European Patent Application EP 4 520 821 A1 - sequence listing, part 14

SEQ ID NO: 18243 - RNA, 5668 nt, Homo sapiens
  source 1..5668: mol_type = other RNA
tgaagtaccagctactcgagaggctgaggcaggagaatcgcatgaacctgggaggcggagcttgcagtgagcggagagtgtgccactgcactccagcctgggcaacaaagcgagactctgtctcaaaaaaaaaaaaaaaaaaaaaacaaagattggattatgatattcagtatctatgtacacatcctatggtgggatggctatccaaaaaaacaagtaaaaagccaaaggtacagataaaatttcatttctgcggaaaagtaaagctcttactgaatggaacagggaagtgagaaactgcagccggcctggccaggcgcggtgccgcagaccctgtcacacagctgctcccagttacgcagcctctccctgtcacccgcagagagcagcatcggtggccgctcagaagccacgacctacaagtaacccttcagacacgttcaaagctcctcgccgagagcctatcaggcttttaagagttggtcattccatgtgaaaagctaattgtgatcttcgaatgtttttctagtccttggctctcattctgctatatattttacttcttgttaaaggcaaaacaaaacttaaatttcatgtcttagaaaaacatcgaccacacaatcaaataaataacattgataagagccttctggggcagcggcgcacggaggcgagtccacagcagtcactctcccggcccttctttggaagccctgctctgactgtgtctctgtgggtcgccgcgtgggccggcgtgaccccccgggggcacagggctggcagtggctggctccagcggcgtccacgaggacagagactcgtgcaccgtcagggcgtgctcctccatctggcgctgcaggctgtccatctcctgcttgagctgctggaggcagctgttcaggttcttgaggggctccttgctcacggcgggcggtggtctcagcagctcctccagcagcgaggcgggaactgggcagtccgggatcttgatgggcgtggcagggttggaagagctggcctcgcctttcggctcctttctcgtcttggccgcgccgcggcgtaggtccagcttgagctgctggttctgctggagcagggtcttcatgttgttcttcagctccgacacttttgcctggagcataaatttatccttctgggtcatggacaggtcttcctgggccatctccaactcagacttgacgttctgcagcagctgctgtagcccttccagttccttcctgccctgctgctccgtcaagtccagctgctgcttcaaggactggatttctctttctttctgatccacctcccatttgagattttccatctcttggtttcccacgggctgtttgctgagctgctcgtccagctgcttctgcaggagctggagctgtgcccgggcctcggccagctctgcttggaactgtgctatctcctgggaatgtttcccctcccgaatctgaaggtcgtcggcctcggcctgcagcttctgcaccaggtgttccttggcctgcagctccttcttcacctcactcagctccaaggaggccgccttgaagtggcggcggttatgcccggcttccaccttggcagcagccacctgctccttgaggctgttcaccttctccttctccttctctagtgaggcctgcagggcctggacaagatgcttcatctggcgatcctcctcttctttgcgctgcaaaactgcctgcacctgaaggttcaactggactaggtctgcctccctcttggccaaagctgtttctaggatgctgttgtgttcccgcagagctgcgttggactgaccgaggcccgtaagcttccctttctcgtgctctaattcaagagccaacttcttgtttgactcctcaaggcgttttatcttcttcctaaagcctctggattcttgaagctcgtcctccagctccagcaccttctcccgggactcctccagctcctggctggtcagcgctatgacctcctgcagttccttttccagcagcgtcttgctatgactgacagcctgcagctccgcctccagggcctggatcctttcatgtagagccaggctgctgtcactgctgccaccctgggctcggagctggcccagctccgcgtccgcagcctccttggccgcgagggcctcctgcaggcggcggctgaggatgcccacggcgttctcgtaggccttatgtttggtcttcatctccttctgggcgctggtcaagtctgagcccagccgcctcatcttctgcttctgttccgtgatggccttccgggcctcttgctgcaactcttcgatttgtttcttcagcgcctcattggcctctgtgaccgcgaccatctgctccttatcgaactgcaacgactgcaagtgtgtttccatctcgtctcgctccttctgcgccgactggagatgcccttcaaggtccgccatgtgctgacggacctgggccacctctctgtgcaggcgcgagagctccgcctcggcagtccgcttctccccgtgcacttgcatcagctcctgccgcagctccttcagctccgagtccagcctcttcctggtggctttcagctcactgatgagctggtctttggaggtggcgtcgcgccggtaggcctccaccatcaccttttgttggagaaactgttcctttattttttgcatttgctttttcagagcagcagtctcctgctgcaggtgttccacctggccggatttgatagctaattcttctcttaacttctctaaagtttccgacgtttcctcggtaccttcttccaagcgtcttgctcctctgtcaagctcctccttgccactcttggccgcctgcaaagccgcctccaagatgatcttctcgttctgcaggaggcagatcgtgtcctccctggaggcggcctcgccctgcagctcccccagcctggcctgcagctcatcgtagtgtgtctgcagggcatcgagggactgctccctgctctgcagagcctcctgagtcaaggtgagctgtttcatcaggtccaggtgctcctgctgcaaagcctcaagctgctggtctcgctggagtaaagtcaacttcacctgctccagctgctgctccagggatgccgccgagtccgccatcctctgcagccgctccctctcaccttcaaactcttccagcctcctctgaaggtcctcctccaccatcgtctttgcctcctgaatctgcatgaaggctgcttcctgatccaacatgtcagcctcaatgccctgcagctgtgccgcgatgcgccccttctccttcatggacctgtgctgagtttccgtcagctgctgggacagggacacattctcgagtttcaggtgctccaggagacctgcctgggtcatctgtccaacctggatgtgggccatctcaccctgcagcctgacgcgggcctcctgtgccagggcgagctgctgctggtaccactgccggacactctgcagggacgagatctccgcctgcgacgccttcagcttgctggtcagcgtcgtccgctccagctgcacctgctgaagctggctctgcaaggctgtcatctgctgtcgcaggtcgtgcactgtgttgtccttgctgagcatgctcctctgcatgtcctctaccttggccataagcctctggtactgctcctcggccacctgcaagtcgttgttggacgacgccaggctggcattttttgcctccagcatgttctgcaggtcagtcatggctcgctccaggtcccagcacgactgcttcagggtgtccacctccgagctcagcgaatcctgccgctgctggctgctgtggctgcactccacctgcgcctgcagcttcgtgctgagggcggccagctgggcctgcagctcagccttctctttaagtgcctgactcgcctccagtgacaaggcttccagctgtccttcgagtcgcattttctctttgagcacctgcagcatctcctcctgtgtttctgctgcagagctctccaaggacacgctgctgcagatgctgtctctccgactccgcacctccccgttgacctcctgcccctggtcttggtgctcagcggctgcggcctggaggacgtccttaatggaggggaactggcccagggtatccgcaggaatctcctggccgttgaccatatagggggtgtcctgcgtgcccactgtcttcgacagaatgccataggtccctcgggtggaggcgctgctgtacgatgagctgtcgctgtcatttccatccacctcagacacgctgtctccagccagggaggtgttctccagacggtcgtcagtgtcgggggacaggctgatctcagacacaacggacgccgcactgcttctgttctgcttcagggaacccttggtagaatcgggagccgggacatttcccccagaattccccgcatttgaatcttcagttctgtaatcggccagagaccggattttgcttgatttggaagtttttttctccctaggatgtgccggaagccccaggctgcccaccttaggcccccgagggacactggtgcgcaggaaggaatattcttttgtcatagccagggtactggcccttggtaagttttctgggtttaacatgagctcaggatcaagcgtgctaaaaagtctcgttttggttgcaggttgactggacctctcctgctggcgcttcaccctgtactgtttgagctgctcttccagccacttccgagcctgaagtcggacctgctcctccttctccaggggcaggggagaatctgtagagcacagttgcgtttcttgcataggaagactgagtctgagagactgcaaagcttcttttctaacactgccctcagcactagttccctgagacttccttaggttgtcatggaaaccagccacacctggagaggcatcagggcccactgggcttgtggtgggatcgagagacgacggagggtctgggaagggtggcgttggcccgttctgacagaggcctccctggccaggtccatccgggctttccccttccgtggatgctctgtttacctcggcacactggactttgtcctgctggtcaggtggcaccagtgggcccgggggcttcagtggggcctcggggagagacgaggggccactgtgggatctgtcctcctggaggccatcttgctcggccgacgcgccgtccatggtcaggacgacaccagctgagctgacgctgaggggctacaagtgaaccttggacaagcttggcttctgccatcagcaacagccaagagctcctgggaggggccctactgtgtctcccattttcaggagaagatctgatgactcacaaatgacttgatgtcaaaccagctaatatcatgatacttgggaaagtatgctacttcttaaggcaatcgggggaaaaaaagctcctcttcaatctgagtgatgtcagatgatttatttccttcttgccatttaaggtatactgcccgtgacaacgcccggccccactcgctctggccacctggaatgaagacaagtcggccagcgacaaagacaaacaaggaagtacacggactcctgaaaccccgacttcccacgaaccacccgacaccatgtcacgcctttcagctgcaaagggccaggctaaagcaagcactgcccgagtggtggcagtggacagct

SEQ ID NO: 18244 - RNA, 5490 nt, Homo sapiens
  source 1..5490: mol_type = other RNA
tgaagtaccagctactcgagaggctgaggcaggagaatcgcatgaacctgggaggcggagcttgcagtgagcggagagtgtgccactgcactccagcctgggcaacaaagcgagactctgtctcaaaaaaaaaaaaaaaaaaaaaacaaagattggattatgatattcagtatctatgtacacatcctatggtgggatggctatccaaaaaaacaagtaaaaagccaaaggtacagataaaatttcatttctgcggaaaagtaaagctcttactgaatggaacagggaagtgagaaactgcagccggcctggccaggcgcggtgccgcagaccctgtcacacagctgctcccagttacgcagcctctccctgtcacccgcagagagcagcatcggtggccgctcagaagccacgacctacaagtaacccttcagacacgttcaaagctcctcgccgagagcctatcaggcttttaagagttggtcattccatgtgaaaagctaattgtgatcttcgaatgtttttctagtccttggctctcattctgctatatattttacttcttgttaaaggcaaaacaaaacttaaatttcatgtcttagaaaaacatcgaccacacaatcaaataaataacattgataagagccttctggggcagcggcgcacggaggcgagtccacagcagtcactctcccggcccttctttggaagccctgctctgactgtgtctctgtgggtcgccgcgtgggccggcgtgaccccccgggggcacagggctggcagtggctggctccagcggcgtccacgaggacagagactcgtgcaccgtcagggcgtgctcctccatctggcgctgcaggctgtccatctcctgcttgagctgctggaggcagctgttcaggttcttgaggggctccttgctcacggcgggcggtggtctcagcagctcctccagcagcgaggcgggaactgggcagtccgggatcttgatgggcgtggcagggttggaagagctggcctcgcctttcggctcctttctcgtcttggccgcgccgcggcgtaggtccagcttgagctgctggttctgctggagcagggtcttcatgttgttcttcagctccgacacttttgcctggagcataaatttatccttctgggtcatggacaggtcttcctgggccatctccaactcagacttgacgttctgcagcagctgctgtagcccttccagttccttcctgccctgctgctccgtcaagtccagctgctgcttcaaggactggatttctctttctttctgatccacctcccatttgagattttccatctcttggtttcccacgggctgtttgctgagctgctcgtccagctgcttctgcaggagctggagctgtgcccgggcctcggccagctctgcttggaactgtgctatctcctgggaatgtttcccctcccgaatctgaaggtcgtcggcctcggcctgcagcttctgcaccaggtgttccttggcctgcagctccttcttcacctcactcagctccaaggaggccgccttgaagtggcggcggttatgcccggcttccaccttggcagcagccacctgctccttgaggctgttcaccttctccttctccttctctagtgaggcctgcagggcctggacaagatgcttcatctggcgatcctcctcttctttgcgctgcaaaactgcctgcacctgaaggttcaactggactaggtctgcctccctcttggccaaagctgtttctaggatgctgttgtgttcccgcagagctgcgttggactgaccgaggcccgtaagcttccctttctcgtgctctaattcaagagccaacttcttgtttgactcctcaaggcgttttatcttcttcctaaagcctctggattcttgaagctcgtcctccagctccagcaccttctcccgggactcctccagctcctggctggtcagcgctatgacctcctgcagttccttttccagcagcgtcttgctatgactgacagcctgcagctccgcctccagggcctggatcctttcatgtagagccaggctgctgtcactgctgccaccctgggctcggagctggcccagctccgcgtccgcagcctccttggccgcgagggcctcctgcaggcggcggctgaggatgcccacggcgttctcgtaggccttatgtttggtcttcatctccttctgggcgctggtcaagtctgagcccagccgcctcatcttctgcttctgttccgtgatggccttccgggcctcttgctgcaactcttcgatttgtttcttcagcgcctcattggcctctgtgaccgcgaccatctgctccttatcgaactgcaacgactgcaagtgtgtttccatctcgtctcgctccttctgcgccgactggagatgcccttcaaggtccgccatgtgctgacggacctgggccacctctctgtgcaggcgcgagagctccgcctcggcagtccgcttctccccgtgcacttgcatcagctcctgccgcagctccttcagctccgagtccagcctcttcctggtggctttcagctcactgatgagctggtctttggaggtggcgtcgcgccggtaggcctccaccatcaccttttgttggagaaactgttcctttattttttgcatttgctttttcagagcagcagtctcctgctgcaggtgttccacctggccggatttgatagctaattcttctcttaacttctctaaagtttccgacgtttcctcggtaccttcttccaagcgtcttgctcctctgtcaagctcctccttgccactcttggccgcctgcaaagccgcctccaagatgatcttctcgttctgcaggaggcagatcgtgtcctccctggaggcggcctcgccctgcagctcccccagcctggcctgcagctcatcgtagtgtgtctgcagggcatcgagggactgctccctgctctgcagagcctcctgagtcaaggtgagctgtttcatcaggtccaggtgctcctgctgcaaagcctcaagctgctggtctcgctggagtaaagtcaacttcacctgctccagctgctgctccagggatgccgccgagtccgccatcctctgcagccgctccctctcaccttcaaactcttccagcctcctctgaaggtcctcctccaccatcgtctttgcctcctgaatctgcatgaaggctgcttcctgatccaacatgtcagcctcaatgccctgcagctgtgccgcgatgcgccccttctccttcatggacctgtgctgagtttccgtcagctgctgggacagggacacattctcgagtttcaggtgctccaggagacctgcctgggtcatctgtccaacctggatgtgggccatctcaccctgcagcctgacgcgggcctcctgtgccagggcgagctgctgctggtaccactgccggacactctgcagggacgagatctccgcctgcgacgccttcagcttgctggtcagcgtcgtccgctccagctgcacctgctgaagctggctctgcaaggctgtcatctgctgtcgcaggtcgtgcactgtgttgtccttgctgagcatgctcctctgcatgtcctctaccttggccataagcctctggtactgctcctcggccacctgcaagtcgttgttggacgacgccaggctggcattttttgcctccagcatgttctgcaggtcagtcatggctcgctccaggtcccagcacgactgcttcagggtgtccacctccgagctcagcgaatcctgccgctgctggctgctgtggctgcactccacctgcgcctgcagcttcgtgctgagggcggccagctgggcctgcagctcagccttctctttaagtgcctgactcgcctccagtgacaaggcttccagctgtccttcgagtcgcattttctctttgagcacctgcagcatctcctcctgtgtttctgctgcagagctctccaaggacacgctgctgcagatgctgtctctccgactccgcacctccccgttgacctcctgcccctggtcttggtgctcagcggctgcggcctggaggacgtccttaatggaggggaactggcccagggtatccgcaggaatctcctggccgttgaccatatagggggtgtcctgcgtgcccactgtcttcgacagaatgccataggtccctcgggtggaggcgctgctgtacgatgagctgtcgctgtcatttccatccacctcagacacgctgtctccagccagggaggtgttctccagacggtcgtcagtgtcgggggacaggctgatctcagacacaacggacgccgcactgcttctgttctgcttcagggaacccttggtagaatcgggagccgggacatttcccccagaattccccgcatttgaatcttcagttctgtaatcggccagagaccggattttgcttgatttggaagtttttttctccctaggatgtgccggaagccccaggctgcccaccttaggcccccgagggacactggtgcgcaggaaggaatattcttttgtcatagccagggtactggcccttggtaagttttctgggtttaacatgagctcaggatcaagcgtgctaaaaagtctcgttttggttgcaggttgactggacctctcctgctggcgcttcaccctgtactgtttgagctgctcttccagccacttccgagcctgaagtcggacctgctcctccttctccaggggcaggggagaatctgtagagcacagttgcgtttcttgcataggaagactgagtctgagagactgcaaagcttcttttctaacactgccctcagcactagttccctgagacttccttaggttgtcatggaaaccagccacacctggagaggcatcagggcccactgggcttgtggtgggatcgagagacgacggagggtctgggaagggtggcgttggcccgttctgacagaggcctccctggccaggtccatccgggctttccccttccgtggatgctctgtttacctcggcacactggactttgtcctgctggtcaggtggcaccagtgggcccgggggcttcagtggggcctcggggagagacgaggggccactgtgggatctgtcctcctggaggccatcttgctcggccgacgcgccgtccatggtcaggacgacaccagctgagctgacgctgaggggctacaagtgaaccttggacaagcttggcttctgccatcagcaacagccaagagctcctgggaggggccctactgtgtctcccattttcaggagaagatctgatgactcacaaatgacttgatgtcaaaccagctaatatcatgatacttgggaaagtatgctacttcttaaggcaatcgggggaaaaaaagctcctcttcaatctgagtgatgtcagatgatttatttccttcttgccatttaaggtatactgccctgctgctctggcagcc

SEQ ID NO: 18245 - RNA, 5515 nt, Homo sapiens
  source 1..5515: mol_type = other RNA
tgaagtaccagctactcgagaggctgaggcaggagaatcgcatgaacctgggaggcggagcttgcagtgagcggagagtgtgccactgcactccagcctgggcaacaaagcgagactctgtctcaaaaaaaaaaaaaaaaaaaaaacaaagattggattatgatattcagtatctatgtacacatcctatggtgggatggctatccaaaaaaacaagtaaaaagccaaaggtacagataaaatttcatttctgcggaaaagtaaagctcttactgaatggaacagggaagtgagaaactgcagccggcctggccaggcgcggtgccgcagaccctgtcacacagctgctcccagttacgcagcctctccctgtcacccgcagagagcagcatcggtggccgctcagaagccacgacctacaagtaacccttcagacacgttcaaagctcctcgccgagagcctatcaggcttttaagagttggtcattccatgtgaaaagctaattgtgatcttcgaatgtttttctagtccttggctctcattctgctatatattttacttcttgttaaaggcaaaacaaaacttaaatttcatgtcttagaaaaacatcgaccacacaatcaaataaataacattgataagagccttctggggcagcggcgcacggaggcgagtccacagcagtcactctcccggcccttctttggaagccctgctctgactgtgtctctgtgggtcgccgcgtgggccggcgtgaccccccgggggcacagggctggcagtggctggctccagcggcgtccacgaggacagagactcgtgcaccgtcagggcgtgctcctccatctggcgctgcaggctgtccatctcctgcttgagctgctggaggcagctgttcaggttcttgaggggctccttgctcacggcgggcggtggtctcagcagctcctccagcagcgaggcgggaactgggcagtccgggatcttgatgggcgtggcagggttggaagagctggcctcgcctttcggctcctttctcgtcttggccgcgccgcggcgtaggtccagcttgagctgctggttctgctggagcagggtcttcatgttgttcttcagctccgacacttttgcctggagcataaatttatccttctgggtcatggacaggtcttcctgggccatctccaactcagacttgacgttctgcagcagctgctgtagcccttccagttccttcctgccctgctgctccgtcaagtccagctgctgcttcaaggactggatttctctttctttctgatccacctcccatttgagattttccatctcttggtttcccacgggctgtttgctgagctgctcgtccagctgcttctgcaggagctggagctgtgcccgggcctcggccagctctgcttggaactgtgctatctcctgggaatgtttcccctcccgaatctgaaggtcgtcggcctcggcctgcagcttctgcaccaggtgttccttggcctgcagctccttcttcacctcactcagctccaaggaggccgccttgaagtggcggcggttatgcccggcttccaccttggcagcagccacctgctccttgaggctgttcaccttctccttctccttctctagtgaggcctgcagggcctggacaagatgcttcatctggcgatcctcctcttctttgcgctgcaaaactgcctgcacctgaaggttcaactggactaggtctgcctccctcttggccaaagctgtttctaggatgctgttgtgttcccgcagagctgcgttggactgaccgaggcccgtaagcttccctttctcgtgctctaattcaagagccaacttcttgtttgactcctcaaggcgttttatcttcttcctaaagcctctggattcttgaagctcgtcctccagctccagcaccttctcccgggactcctccagctcctggctggtcagcgctatgacctcctgcagttccttttccagcagcgtcttgctatgactgacagcctgcagctccgcctccagggcctggatcctttcatgtagagccaggctgctgtcactgctgccaccctgggctcggagctggcccagctccgcgtccgcagcctccttggccgcgagggcctcctgcaggcggcggctgaggatgcccacggcgttctcgtaggccttatgtttggtcttcatctccttctgggcgctggtcaagtctgagcccagccgcctcatcttctgcttctgttccgtgatggccttccgggcctcttgctgcaactcttcgatttgtttcttcagcgcctcattggcctctgtgaccgcgaccatctgctccttatcgaactgcaacgactgcaagtgtgtttccatctcgtctcgctccttctgcgccgactggagatgcccttcaaggtccgccatgtgctgacggacctgggccacctctctgtgcaggcgcgagagctccgcctcggcagtccgcttctccccgtgcacttgcatcagctcctgccgcagctccttcagctccgagtccagcctcttcctggtggctttcagctcactgatgagctggtctttggaggtggcgtcgcgccggtaggcctccaccatcaccttttgttggagaaactgttcctttattttttgcatttgctttttcagagcagcagtctcctgctgcaggtgttccacctggccggatttgatagctaattcttctcttaacttctctaaagtttccgacgtttcctcggtaccttcttccaagcgtcttgctcctctgtcaagctcctccttgccactcttggccgcctgcaaagccgcctccaagatgatcttctcgttctgcaggaggcagatcgtgtcctccctggaggcggcctcgccctgcagctcccccagcctggcctgcagctcatcgtagtgtgtctgcagggcatcgagggactgctccctgctctgcagagcctcctgagtcaaggtgagctgtttcatcaggtccaggtgctcctgctgcaaagcctcaagctgctggtctcgctggagtaaagtcaacttcacctgctccagctgctgctccagggatgccgccgagtccgccatcctctgcagccgctccctctcaccttcaaactcttccagcctcctctgaaggtcctcctccaccatcgtctttgcctcctgaatctgcatgaaggctgcttcctgatccaacatgtcagcctcaatgccctgcagctgtgccgcgatgcgccccttctccttcatggacctgtgctgagtttccgtcagctgctgggacagggacacattctcgagtttcaggtgctccaggagacctgcctgggtcatctgtccaacctggatgtgggccatctcaccctgcagcctgacgcgggcctcctgtgccagggcgagctgctgctggtaccactgccggacactctgcagggacgagatctccgcctgcgacgccttcagcttgctggtcagcgtcgtccgctccagctgcacctgctgaagctggctctgcaaggctgtcatctgctgtcgcaggtcgtgcactgtgttgtccttgctgagcatgctcctctgcatgtcctctaccttggccataagcctctggtactgctcctcggccacctgcaagtcgttgttggacgacgccaggctggcattttttgcctccagcatgttctgcaggtcagtcatggctcgctccaggtcccagcacgactgcttcagggtgtccacctccgagctcagcgaatcctgccgctgctggctgctgtggctgcactccacctgcgcctgcagcttcgtgctgagggcggccagctgggcctgcagctcagccttctctttaagtgcctgactcgcctccagtgacaaggcttccagctgtccttcgagtcgcattttctctttgagcacctgcagcatctcctcctgtgtttctgctgcagagctctccaaggacacgctgctgcagatgctgtctctccgactccgcacctccccgttgacctcctgcccctggtcttggtgctcagcggctgcggcctggaggacgtccttaatggaggggaactggcccagggtatccgcaggaatctcctggccgttgaccatatagggggtgtcctgcgtgcccactgtcttcgacagaatgccataggtccctcgggtggaggcgctgctgtacgatgagctgtcgctgtcatttccatccacctcagacacgctgtctccagccagggaggtgttctccagacggtcgtcagtgtcgggggacaggctgatctcagacacaacggacgccgcactgcttctgttctgcttcagggaacccttggtagaatcgggagccgggacatttcccccagaattccccgcatttgaatcttcagttctgtaatcggccagagaccggattttgcttgatttggaagtttttttctccctaggatgtgccggaagccccaggctgcccaccttaggcccccgagggacactggtgcgcaggaaggaatattcttttgtcatagccagggtactggcccttggtaagttttctgggtttaacatgagctcaggatcaagcgtgctaaaaagtctcgttttggttgcaggttgactggacctctcctgctggcgcttcaccctgtactgtttgagctgctcttccagccacttccgagcctgaagtcggacctgctcctccttctccaggggcaggggagaatctgtagagcacagttgcgtttcttgcataggaagactgagtctgagagactgcaaagcttcttttctaacactgccctcagcactagttccctgagacttccttaggttgtcatggaaaccagccacacctggagaggcatcagggcccactgggcttgtggtgggatcgagagacgacggagggtctgggaagggtggcgttggcccgttctgacagaggcctccctggccaggtccatccgggctttccccttccgtggatgctctgtttacctcggcacactggactttgtcctgctggtcaggtggcaccagtgggcccgggggcttcagtggggcctcggggagagacgaggggccactgtgggatctgtcctcctggaggccatcttgctcggccgacgcgccgtccatggtcaggacgacaccagctgagctgacgctgaggggctacaagtgaaccttggacaagcttggcttctgccatcagcaacagccaagagctcctgggaggggccctactgtgtctcccattttcaggagaagatctgatgactcacaaatgacttgatgtcaaaccagctaatatcatgatacttgggaaagtatgctacttcttaaggcaatcgggggaaaaaaagctcctcttcaatctgagtgatgtcagatgatttatttccttcttgccatttaaggtatactgcctgtaacaccagcactttgggaggctggggtgggaggatcgct

SEQ ID NO: 18246 - RNA, 5195 nt, Homo sapiens
  source 1..5195: mol_type = other RNA
tgaagtaccagctactcgagaggctgaggcaggagaatcgcatgaacctgggaggcggagcttgcagtgagcggagagtgtgccactgcactccagcctgggcaacaaagcgagactctgtctcaaaaaaaaaaaaaaaaaaaaaacaaagattggattatgatattcagtatctatgtacacatcctatggtgggatggctatccaaaaaaacaagtaaaaagccaaaggtacagataaaatttcatttctgcggaaaagtaaagctcttactgaatggaacagggaagtgagaaactgcagccggcctggccaggcgcggtgccgcagaccctgtcacacagctgctcccagttacgcagcctctccctgtcacccgcagagagcagcatcggtggccgctcagaagccacgacctacaagtaacccttcagacacgttcaaagctcctcgccgagagcctatcaggcttttaagagttggtcattccatgtgaaaagctaattgtgatcttcgaatgtttttctagtccttggctctcattctgctatatattttacttcttgttaaaggcaaaacaaaacttaaatttcatgtcttagaaaaacatcgaccacacaatcaaataaataacattgataagagccttctggggcagcggcgcacggaggcgagtccacagcagtcactctcccggcccttctttggaagccctgctctgactgtgtctctgtgggtcgccgcgtgggccggcgtgaccccccgggggcacagggctggcagtggctggctccagcggcgtccacgaggacagagactcgtgcaccgtcagggcgtgctcctccatctggcgctgcaggctgtccatctcctgcttgagctgctggaggcagctgttcaggttcttgaggggctccttgctcacggcgggcggtggtctcagcagctcctccagcagcgaggcgggaactgggcagtccgggatcttgatgggcgtggcagggttggaagagctggcctcgcctttcggctcctttctcgtcttggccgcgccgcggcgtaggtccagcttgagctgctggttctgctggagcagggtcttcatgttgttcttcagctccgacacttttgcctggagcataaatttatccttctgggtcatggacaggtcttcctgggccatctccaactcagacttgacgttctgcagcagctgctgtagcccttccagttccttcctgccctgctgctccgtcaagtccagctgctgcttcaaggactggatttctctttctttctgatccacctcccatttgagattttccatctcttggtttcccacgggctgtttgctgagctgctcgtccagctgcttctgcaggagctggagctgtgcccgggcctcggccagctctgcttggaactgtgctatctcctgggaatgtttcccctcccgaatctgaaggtcgtcggcctcggcctgcagcttctgcaccaggtgttccttggcctgcagctccttcttcacctcactcagctccaaggaggccgccttgaagtggcggcggttatgcccggcttccaccttggcagcagccacctgctccttgaggctgttcaccttctccttctccttctctagtgaggcctgcagggcctggacaagatgcttcatctggcgatcctcctcttctttgcgctgcaaaactgcctgcacctgaaggttcaactggactaggtctgcctccctcttggccaaagctgtttctaggatgctgttgtgttcccgcagagctgcgttggactgaccgaggcccgtaagcttccctttctcgtgctctaattcaagagccaacttcttgtttgactcctcaaggcgttttatcttcttcctaaagcctctggattcttgaagctcgtcctccagctccagcaccttctcccgggactcctccagctcctggctggtcagcgctatgacctcctgcagttccttttccagcagcgtcttgctatgactgacagcctgcagctccgcctccagggcctggatcctttcatgtagagccaggctgctgtcactgctgccaccctgggctcggagctggcccagctccgcgtccgcagcctccttggccgcgagggcctcctgcaggcggcggctgaggatgcccacggcgttctcgtaggccttatgtttggtcttcatctccttctgggcgctggtcaagtctgagcccagccgcctcatcttctgcttctgttccgtgatggccttccgggcctcttgctgcaactcttcgatttgtttcttcagcgcctcattggcctctgtgaccgcgaccatctgctccttatcgaactgcaacgactgcaagtgtgtttccatctcgtctcgctccttctgcgccgactggagatgcccttcaaggtccgccatgtgctgacggacctgggccacctctctgtgcaggcgcgagagctccgcctcggcagtccgcttctccccgtgcacttgcatcagctcctgccgcagctccttcagctccgagtccagcctcttcctggtggctttcagctcactgatgagctggtctttggaggtggcgtcgcgccggtaggcctccaccatcaccttttgttggagaaactgttcctttattttttgcatttgctttttcagagcagcagtctcctgctgcaggtgttccacctggccggatttgatagctaattcttctcttaacttctctaaagtttccgacgtttcctcggtaccttcttccaagcgtcttgctcctctgtcaagctcctccttgccactcttggccgcctgcaaagccgcctccaagatgatcttctcgttctgcaggaggcagatcgtgtcctccctggaggcggcctcgccctgcagctcccccagcctggcctgcagctcatcgtagtgtgtctgcagggcatcgagggactgctccctgctctgcagagcctcctgagtcaaggtgagctgtttcatcaggtccaggtgctcctgctgcaaagcctcaagctgctggtctcgctggagtaaagtcaacttcacctgctccagctgctgctccagggatgccgccgagtccgccatcctctgcagccgctccctctcaccttcaaactcttccagcctcctctgaaggtcctcctccaccatcgtctttgcctcctgaatctgcatgaaggctgcttcctgatccaacatgtcagcctcaatgccctgcagctgtgccgcgatgcgccccttctccttcatggacctgtgctgagtttccgtcagctgctgggacagggacacattctcgagtttcaggtgctccaggagacctgcctgggtcatctgtccaacctggatgtgggccatctcaccctgcagcctgacgcgggcctcctgtgccagggcgagctgctgctggtaccactgccggacactctgcagggacgagatctccgcctgcgacgccttcagcttgctggtcagcgtcgtccgctccagctgcacctgctgaagctggctctgcaaggctgtcatctgctgtcgcaggtcgtgcactgtgttgtccttgctgagcatgctcctctgcatgtcctctaccttggccataagcctctggtactgctcctcggccacctgcaagtcgttgttggacgacgccaggctggcattttttgcctccagcatgttctgcaggtcagtcatggctcgctccaggtcccagcacgactgcttcagggtgtccacctccgagctcagcgaatcctgccgctgctggctgctgtggctgcactccacctgcgcctgcagcttcgtgctgagggcggccagctgggcctgcagctcagccttctctttaagtgcctgactcgcctccagtgacaaggcttccagctgtccttcgagtcgcattttctctttgagcacctgcagcatctcctcctgtgtttctgctgcagagctctccaaggacacgctgctgcagatgctgtctctccgactccgcacctccccgttgacctcctgcccctggtcttggtgctcagcggctgcggcctggaggacgtccttaatggaggggaactggcccagggtatccgcaggaatctcctggccgttgaccatatagggggtgtcctgcgtgcccactgtcttcgacagaatgccataggtccctcgggtggaggcgctgctgtacgatgagctgtcgctgtcatttccatccacctcagacacgctgtctccagccagggaggtgttctccagacggtcgtcagtgtcgggggacaggctgatctcagacacaacggacgccgcactgcttctgttctgcttcagggaacccttggtagaatcgggagccgggacatttcccccagaattccccgcatttgaatcttcagttctgtaatcggccagagaccggattttgcttgatttggaagtttttttctccctaggatgtgccggaagccccaggctgcccaccttaggcccccgagggacactggtgcgcaggaaggaatattcttttgtcatagccagggtactggcccttggtaagttttctgggtttaacatgagctcaggatcaagcgtgctaaaaagtctcgttttggttgcaggttgactggacctctcctgctggcgcttcaccctgtactgtttgagctgctcttccagccacttccgagcctgaagtcggacctgctcctccttctccaggggcaggggagaatctgtagagcactggactttgtcctgctggtcaggtggcaccagtgggcccgggggcttcagtggggcctcggggagagacgaggggccactgtgggatctgtcctcctggaggccatcttgctcggccgacgcgccgtccatggtcaggacgacaccagctgagctgacgctgaggggctacaagtgaaccttggacaagcttggcttctgccatcagcaacagccaagagctcctgggaggggccctactgtgtctcccattttcaggagaagatctgatgactcacaaatgacttgatgtcaaaccagctaatatcatgataccctgctgctctggcagccccggaggccgcccggcccggatgctccggcggagacgtggccgtgagaggggcggggcgagcggtgcatcggcctcgggtccccg

SEQ ID NO: 18247 - RNA, 5348 nt, Homo sapiens
  source 1..5348: mol_type = other RNA
tgaagtaccagctactcgagaggctgaggcaggagaatcgcatgaacctgggaggcggagcttgcagtgagcggagagtgtgccactgcactccagcctgggcaacaaagcgagactctgtctcaaaaaaaaaaaaaaaaaaaaaacaaagattggattatgatattcagtatctatgtacacatcctatggtgggatggctatccaaaaaaacaagtaaaaagccaaaggtacagataaaatttcatttctgcggaaaagtaaagctcttactgaatggaacagggaagtgagaaactgcagccggcctggccaggcgcggtgccgcagaccctgtcacacagctgctcccagttacgcagcctctccctgtcacccgcagagagcagcatcggtggccgctcagaagccacgacctacaagtaacccttcagacacgttcaaagctcctcgccgagagcctatcaggcttttaagagttggtcattccatgtgaaaagctaattgtgatcttcgaatgtttttctagtccttggctctcattctgctatatattttacttcttgttaaaggcaaaacaaaacttaaatttcatgtcttagaaaaacatcgaccacacaatcaaataaataacattgataagagccttctggggcagcggcgcacggaggcgagtccacagcagtcactctcccggcccttctttggaagccctgctctgactgtgtctctgtgggtcgccgcgtgggccggcgtgaccccccgggggcacagggctggcagtggctggctccagcggcgtccacgaggacagagactcgtgcaccgtcagggcgtgctcctccatctggcgctgcaggctgtccatctcctgcttgagctgctggaggcagctgttcaggttcttgaggggctccttgctcacggcgggcggtggtctcagcagctcctccagcagcgaggcgggaactgggcagtccgggatcttgatgggcgtggcagggttggaagagctggcctcgcctttcggctcctttctcgtcttggccgcgccgcggcgtaggtccagcttgagctgctggttctgctggagcagggtcttcatgttgttcttcagctccgacacttttgcctggagcataaatttatccttctgggtcatggacaggtcttcctgggccatctccaactcagacttgacgttctgcagcagctgctgtagcccttccagttccttcctgccctgctgctccgtcaagtccagctgctgcttcaaggactggatttctctttctttctgatccacctcccatttgagattttccatctcttggtttcccacgggctgtttgctgagctgctcgtccagctgcttctgcaggagctggagctgtgcccgggcctcggccagctctgcttggaactgtgctatctcctgggaatgtttcccctcccgaatctgaaggtcgtcggcctcggcctgcagcttctgcaccaggtgttccttggcctgcagctccttcttcacctcactcagctccaaggaggccgccttgaagtggcggcggttatgcccggcttccaccttggcagcagccacctgctccttgaggctgttcaccttctccttctccttctctagtgaggcctgcagggcctggacaagatgcttcatctggcgatcctcctcttctttgcgctgcaaaactgcctgcacctgaaggttcaactggactaggtctgcctccctcttggccaaagctgtttctaggatgctgttgtgttcccgcagagctgcgttggactgaccgaggcccgtaagcttccctttctcgtgctctaattcaagagccaacttcttgtttgactcctcaaggcgttttatcttcttcctaaagcctctggattcttgaagctcgtcctccagctccagcaccttctcccgggactcctccagctcctggctggtcagcgctatgacctcctgcagttccttttccagcagcgtcttgctatgactgacagcctgcagctccgcctccagggcctggatcctttcatgtagagccaggctgctgtcactgctgccaccctgggctcggagctggcccagctccgcgtccgcagcctccttggccgcgagggcctcctgcaggcggcggctgaggatgcccacggcgttctcgtaggccttatgtttggtcttcatctccttctgggcgctggtcaagtctgagcccagccgcctcatcttctgcttctgttccgtgatggccttccgggcctcttgctgcaactcttcgatttgtttcttcagcgcctcattggcctctgtgaccgcgaccatctgctccttatcgaactgcaacgactgcaagtgtgtttccatctcgtctcgctccttctgcgccgactggagatgcccttcaaggtccgccatgtgctgacggacctgggccacctctctgtgcaggcgcgagagctccgcctcggcagtccgcttctccccgtgcacttgcatcagctcctgccgcagctccttcagctccgagtccagcctcttcctggtggctttcagctcactgatgagctggtctttggaggtggcgtcgcgccggtaggcctccaccatcaccttttgttggagaaactgttcctttattttttgcatttgctttttcagagcagcagtctcctgctgcaggtgttccacctggccggatttgatagctaattcttctcttaacttctctaaagtttccgacgtttcctcggtaccttcttccaagcgtcttgctcctctgtcaagctcctccttgccactcttggccgcctgcaaagccgcctccaagatgatcttctcgttctgcaggaggcagatcgtgtcctccctggaggcggcctcgccctgcagctcccccagcctggcctgcagctcatcgtagtgtgtctgcagggcatcgagggactgctccctgctctgcagagcctcctgagtcaaggtgagctgtttcatcaggtccaggtgctcctgctgcaaagcctcaagctgctggtctcgctggagtaaagtcaacttcacctgctccagctgctgctccagggatgccgccgagtccgccatcctctgcagccgctccctctcaccttcaaactcttccagcctcctctgaaggtcctcctccaccatcgtctttgcctcctgaatctgcatgaaggctgcttcctgatccaacatgtcagcctcaatgccctgcagctgtgccgcgatgcgccccttctccttcatggacctgtgctgagtttccgtcagctgctgggacagggacacattctcgagtttcaggtgctccaggagacctgcctgggtcatctgtccaacctggatgtgggccatctcaccctgcagcctgacgcgggcctcctgtgccagggcgagctgctgctggtaccactgccggacactctgcagggacgagatctccgcctgcgacgccttcagcttgctggtcagcgtcgtccgctccagctgcacctgctgaagctggctctgcaaggctgtcatctgctgtcgcaggtcgtgcactgtgttgtccttgctgagcatgctcctctgcatgtcctctaccttggccataagcctctggtactgctcctcggccacctgcaagtcgttgttggacgacgccaggctggcattttttgcctccagcatgttctgcaggtcagtcatggctcgctccaggtcccagcacgactgcttcagggtgtccacctccgagctcagcgaatcctgccgctgctggctgctgtggctgcactccacctgcgcctgcagcttcgtgctgagggcggccagctgggcctgcagctcagccttctctttaagtgcctgactcgcctccagtgacaaggcttccagctgtccttcgagtcgcattttctctttgagcacctgcagcatctcctcctgtgtttctgctgcagagctctccaaggacacgctgctgcagatgctgtctctccgactccgcacctccccgttgacctcctgcccctggtcttggtgctcagcggctgcggcctggaggacgtccttaatggaggggaactggcccagggtatccgcaggaatctcctggccgttgaccatatagggggtgtcctgcgtgcccactgtcttcgacagaatgccataggtccctcgggtggaggcgctgctgtacgatgagctgtcgctgtcatttccatccacctcagacacgctgtctccagccagggaggtgttctccagacggtcgtcagtgtcgggggacaggctgatctcagacacaacggacgccgcactgcttctgttctgcttcagggaacccttggtagaatcgggagccgggacatttcccccagaattccccgcatttgaatcttcagttctgtaatcggccagagaccggattttgcttgatttggaagtttttttctccctaggatgtgccggaagccccaggctgcccaccttaggcccccgagggacactggtgcgcaggaaggaatattcttttgtcatagccagggtactggcccttggtaagttttctgggtttaacatgagctcaggatcaagcgtgctaaaaagtctcgttttggttgcaggttgactggacctctcctgctggcgcttcaccctgtactgtttgagctgctcttccagccacttccgagcctgaagtcggacctgctcctccttctccaggggcaggggagaatctgtagagcctggagaggcatcagggcccactgggcttgtggtgggatcgagagacgacggagggtctgggaagggtggcgttggcccgttctgacagaggcctccctggccaggtccatccgggctttccccttccgtggatgctctgtttacctcggcacactggactttgtcctgctggtcaggtggcaccagtgggcccgggggcttcagtggggcctcggggagagacgaggggccactgtgggatctgtcctcctggaggccatcttgctcggccgacgcgccgtccatggtcaggacgacaccagctgagctgacgctgaggggctacaagtgaaccttggacaagcttggcttctgccatcagcaacagccaagagctcctgggaggggccctactgtgtctcccattttcaggagaagatctgatgactcacaaatgacttgatgtcaaaccagctaatatcatgataccctgctgctctggcagccccggaggccgcccggcccggatgctccggcggagacgtggccgtgagaggggcggggcgagcggtgcatcggcctcgggtccccg

SEQ ID NO: 18248 - RNA, 5358 nt, Homo sapiens
  source 1..5358: mol_type = other RNA
tgaagtaccagctactcgagaggctgaggcaggagaatcgcatgaacctgggaggcggagcttgcagtgagcggagagtgtgccactgcactccagcctgggcaacaaagcgagactctgtctcaaaaaaaaaaaaaaaaaaaaaacaaagattggattatgatattcagtatctatgtacacatcctatggtgggatggctatccaaaaaaacaagtaaaaagccaaaggtacagataaaatttcatttctgcggaaaagtaaagctcttactgaatggaacagggaagtgagaaactgcagccggcctggccaggcgcggtgccgcagaccctgtcacacagctgctcccagttacgcagcctctccctgtcacccgcagagagcagcatcggtggccgctcagaagccacgacctacaagtaacccttcagacacgttcaaagctcctcgccgagagcctatcaggcttttaagagttggtcattccatgtgaaaagctaattgtgatcttcgaatgtttttctagtccttggctctcattctgctatatattttacttcttgttaaaggcaaaacaaaacttaaatttcatgtcttagaaaaacatcgaccacacaatcaaataaataacattgataagagccttctggggcagcggcgcacggaggcgagtccacagcagtcactctcccggcccttctttggaagccctgctctgactgtgtctctgtgggtcgccgcgtgggccggcgtgaccccccgggggcacagggctggcagtggctggctccagcggcgtccacgaggacagagactcgtgcaccgtcagggcgtgctcctccatctggcgctgcaggctgtccatctcctgcttgagctgctggaggcagctgttcaggttcttgaggggctccttgctcacggcgggcggtggtctcagcagctcctccagcagcgaggcgggaactgggcagtccgggatcttgatgggcgtggcagggttggaagagctggcctcgcctttcggctcctttctcgtcttggccgcgccgcggcgtaggtccagcttgagctgctggttctgctggagcagggtcttcatgttgttcttcagctccgacacttttgcctggagcataaatttatccttctgggtcatggacaggtcttcctgggccatctccaactcagacttgacgttctgcagcagctgctgtagcccttccagttccttcctgccctgctgctccgtcaagtccagctgctgcttcaaggactggatttctctttctttctgatccacctcccatttgagattttccatctcttggtttcccacgggctgtttgctgagctgctcgtccagctgcttctgcaggagctggagctgtgcccgggcctcggccagctctgcttggaactgtgctatctcctgggaatgtttcccctcccgaatctgaaggtcgtcggcctcggcctgcagcttctgcaccaggtgttccttggcctgcagctccttcttcacctcactcagctccaaggaggccgccttgaagtggcggcggttatgcccggcttccaccttggcagcagccacctgctccttgaggctgttcaccttctccttctccttctctagtgaggcctgcagggcctggacaagatgcttcatctggcgatcctcctcttctttgcgctgcaaaactgcctgcacctgaaggttcaactggactaggtctgcctccctcttggccaaagctgtttctaggatgctgttgtgttcccgcagagctgcgttggactgaccgaggcccgtaagcttccctttctcgtgctctaattcaagagccaacttcttgtttgactcctcaaggcgttttatcttcttcctaaagcctctggattcttgaagctcgtcctccagctccagcaccttctcccgggactcctccagctcctggctggtcagcgctatgacctcctgcagttccttttccagcagcgtcttgctatgactgacagcctgcagctccgcctccagggcctggatcctttcatgtagagccaggctgctgtcactgctgccaccctgggctcggagctggcccagctccgcgtccgcagcctccttggccgcgagggcctcctgcaggcggcggctgaggatgcccacggcgttctcgtaggccttatgtttggtcttcatctccttctgggcgctggtcaagtctgagcccagccgcctcatcttctgcttctgttccgtgatggccttccgggcctcttgctgcaactcttcgatttgtttcttcagcgcctcattggcctctgtgaccgcgaccatctgctccttatcgaactgcaacgactgcaagtgtgtttccatctcgtctcgctccttctgcgccgactggagatgcccttcaaggtccgccatgtgctgacggacctgggccacctctctgtgcaggcgcgagagctccgcctcggcagtccgcttctccccgtgcacttgcatcagctcctgccgcagctccttcagctccgagtccagcctcttcctggtggctttcagctcactgatgagctggtctttggaggtggcgtcgcgccggtaggcctccaccatcaccttttgttggagaaactgttcctttattttttgcatttgctttttcagagcagcagtctcctgctgcaggtgttccacctggccggatttgatagctaattcttctcttaacttctctaaagtttccgacgtttcctcggtaccttcttccaagcgtcttgctcctctgtcaagctcctccttgccactcttggccgcctgcaaagccgcctccaagatgatcttctcgttctgcaggaggcagatcgtgtcctccctggaggcggcctcgccctgcagctcccccagcctggcctgcagctcatcgtagtgtgtctgcagggcatcgagggactgctccctgctctgcagagcctcctgagtcaaggtgagctgtttcatcaggtccaggtgctcctgctgcaaagcctcaagctgctggtctcgctggagtaaagtcaacttcacctgctccagctgctgctccagggatgccgccgagtccgccatcctctgcagccgctccctctcaccttcaaactcttccagcctcctctgaaggtcctcctccaccatcgtctttgcctcctgaatctgcatgaaggctgcttcctgatccaacatgtcagcctcaatgccctgcagctgtgccgcgatgcgccccttctccttcatggacctgtgctgagtttccgtcagctgctgggacagggacacattctcgagtttcaggtgctccaggagacctgcctgggtcatctgtccaacctggatgtgggccatctcaccctgcagcctgacgcgggcctcctgtgccagggcgagctgctgctggtaccactgccggacactctgcagggacgagatctccgcctgcgacgccttcagcttgctggtcagcgtcgtccgctccagctgcacctgctgaagctggctctgcaaggctgtcatctgctgtcgcaggtcgtgcactgtgttgtccttgctgagcatgctcctctgcatgtcctctaccttggccataagcctctggtactgctcctcggccacctgcaagtcgttgttggacgacgccaggctggcattttttgcctccagcatgttctgcaggtcagtcatggctcgctccaggtcccagcacgactgcttcagggtgtccacctccgagctcagcgaatcctgccgctgctggctgctgtggctgcactccacctgcgcctgcagcttcgtgctgagggcggccagctgggcctgcagctcagccttctctttaagtgcctgactcgcctccagtgacaaggcttccagctgtccttcgagtcgcattttctctttgagcacctgcagcatctcctcctgtgtttctgctgcagagctctccaaggacacgctgctgcagatgctgtctctccgactccgcacctccccgttgacctcctgcccctggtcttggtgctcagcggctgcggcctggaggacgtccttaatggaggggaactggcccagggtatccgcaggaatctcctggccgttgaccatatagggggtgtcctgcgtgcccactgtcttcgacagaatgccataggtccctcgggtggaggcgctgctgtacgatgagctgtcgctgtcatttccatccacctcagacacgctgtctccagccagggaggtgttctccagacggtcgtcagtgtcgggggacaggctgatctcagacacaacggacgccgcactgcttctgttctgcttcagggaacccttggtagaatcgggagccgggacatttcccccagaattccccgcatttgaatcttcagttctgtaatcggccagagaccggattttgcttgatttggaagtttttttctccctaggatgtgccggaagccccaggctgcccaccttaggcccccgagggacactggtgcgcaggaaggaatattcttttgtcatagccagggtactggcccttggtaagttttctgggtttaacatgagctcaggatcaagcgtgctaaaaagtctcgttttggttgcaggttgactggacctctcctgctggcgcttcaccctgtactgtttgagctgctcttccagccacttccgagcctgaagtcggacctgctcctccttctccaggggcaggggagaatctgtagagcctggagaggcatcagggcccactgggcttgtggtgggatcgagagacgacggagggtctgggaagggtggcgttggcccgttctgacagaggcctccctggccaggtccatccgggctttccccttccgtggatgctctgtttacctcggcacactggactttgtcctgctggtcaggtggcaccagtgggcccgggggcttcagtggggcctcggggagagacgaggggccactgtgggatctgtcctcctggaggccatcttgctcggccgacgcgccgtccatggtcaggacgacaccagctgagctgacgctgaggggctacaagtgaaccttggacaagcttggcttctgccatcagcaacagccaagagctcctgggaggggccctactgtgtctcccattttcaggagaagatctgatgactcacaaatgacttgatgtcaaaccagctaatatcatgatacctccgactgtgatgaggccgccttcagaaagtgaccttaagagtttgcggacctttccctagtagaaacgcaacttccggaactgcaggaccaactctttcaggaagctgaac

SEQ ID NO: 18249 - RNA, 4773 nt, Homo sapiens
  source 1..4773: mol_type = other RNA
tgaagtaccagctactcgagaggctgaggcaggagaatcgcatgaacctgggaggcggagcttgcagtgagcggagagtgtgccactgcactccagcctgggcaacaaagcgagactctgtctcaaaaaaaaaaaaaaaaaaaaaacaaagattggattatgatattcagtatctatgtacacatcctatggtgggatggctatccaaaaaaacaagtaaaaagccaaaggtacagataaaatttcatttctgcggaaaagtaaagctcttactgaatggaacagggaagtgagaaactgcagccggcctggccaggcgcggtgccgcagaccctgtcacacagctgctcccagttacgcagcctctccctgtcacccgcagagagcagcatcggtggccgctcagaagccacgacctacaagtaacccttcagacacgttcaaagctcctcgccgagagcctatcaggcttttaagagttggtcattccatgtgaaaagctaattgtgatcttcgaatgtttttctagtccttggctctcattctgctatatattttacttcttgttaaaggcaaaacaaaacttaaatttcatgtcttagaaaaacatcgaccacacaatcaaataaataacattgataagagccttctggggcagcggcgcacggaggcgagtccacagcagtcactctcccggcccttctttggaagccctgctctgactgtgtctctgtgggtcgccgcgtgggccggcgtgaccccccgggggcacagggctggcagtggctggctccagcggcgtccacgaggacagagactcgtgcaccgtcagggcgtgctcctccatctggcgctgcaggctgtccatctcctgcttgagctgctggaggcagctgttcaggttcttgaggggctccttgctcacggcgggcggtggtctcagcagctcctccagcagcgaggcgggaactgggcagtccgggatcttgatgggcgtggcagggttggaagagctggcctcgcctttcggctcctttctcgtcttggccgcgccgcggcgtaggtccagcttgagctgctggttctgctggagcagggtcttcatgttgttcttcagctccgacacttttgcctggagcataaatttatccttctgggtcatggacaggtcttcctgggccatctccaactcagacttgacgttctgcagcagctgctgtagcccttccagttccttcctgccctgctgctccgtcaagtccagctgctgcttcaaggactggatttctctttctttctgatccacctcccatttgagattttccatctcttggtttcccacgggctgtttgctgagctgctcgtccagctgcttctgcaggagctggagctgtgcccgggcctcggccagctctgcttggaactgtgctatctcctgggaatgtttcccctcccgaatctgaaggtcgtcggcctcggcctgcagcttctgcaccaggtgttccttggcctgcagctccttcttcacctcactcagctccaaggaggccgccttgaagtggcggcggttatgcccggcttccaccttggcagcagccacctgctccttgaggctgttcaccttctccttctccttctctagtgaggcctgcagggcctggacaagatgcttcatctggcgatcctcctcttctttgcgctgcaaaactgcctgcacctgaaggttcaactggactaggtctgcctccctcttggccaaagctgtttctaggatgctgttgtgttcccgcagagctgcgttggactgaccgaggcccgtaagcttccctttctcgtgctctaattcaagagccaacttcttgtttgactcctcaaggcgttttatcttcttcctaaagcctctggattcttgaagctcgtcctccagctccagcaccttctcccgggactcctccagctcctggctggtcagcgctatgacctcctgcagttccttttccagcagcgtcttgctatgactgacagcctgcagctccgcctccagggcctggatcctttcatgtagagccaggctgctgtcactgctgccaccctgggctcggagctggcccagctccgcgtccgcagcctccttggccgcgagggcctcctgcaggcggcggctgaggatgcccacggcgttctcgtaggccttatgtttggtcttcatctccttctgggcgctggtcaagtctgagcccagccgcctcatcttctgcttctgttccgtgatggccttccgggcctcttgctgcaactcttcgatttgtttcttcagcgcctcattggcctctgtgaccgcgaccatctgctccttatcgaactgcaacgactgcaagtgtgtttccatctcgtctcgctccttctgcgccgactggagatgcccttcaaggtccgccatgtgctgacggacctgggccacctctctgtgcaggcgcgagagctccgcctcggcagtccgcttctccccgtgcacttgcatcagctcctgccgcagctccttcagctccgagtccagcctcttcctggtggctttcagctcactgatgagctggtctttggaggtggcgtcgcgccggtaggcctccaccatcaccttttgttggagaaactgttcctttattttttgcatttgctttttcagagcagcagtctcctgctgcaggtgttccacctggccggatttgatagctaattcttctcttaacttctctaaagtttccgacgtttcctcggtaccttcttccaagcgtcttgctcctctgtcaagctcctccttgccactcttggccgcctgcaaagccgcctccaagatgatcttctcgttctgcaggaggcagatcgtgtcctccctggaggcggcctcgccctgcagctcccccagcctggcctgcagctcatcgtagtgtgtctgcagggcatcgagggactgctccctgctctgcagagcctcctgagtcaaggtgagctgtttcatcaggtccaggtgctcctgctgcaaagcctcaagctgctggtctcgctggagtaaagtcaacttcacctgctccagctgctgctccagggatgccgccgagtccgccatcctctgcagccgctccctctcaccttcaaactcttccagcctcctctgaaggtcctcctccaccatcgtctttgcctcctgaatctgcatgaaggctgcttcctgatccaacatgtcagcctcaatgccctgcagctgtgccgcgatgcgccccttctccttcatggacctgtgctgagtttccgtcagctgctgggacagggacacattctcgagtttcaggtgctccaggagacctgcctgggtcatctgtccaacctggatgtgggccatctcaccctgcagcctgacgcgggcctcctgtgccagggcgagctgctgctggtaccactgccggacactctgcagggacgagatctccgcctgcgacgccttcagcttgctggtcagcgtcgtccgctccagctgcacctgctgaagctggctctgcaaggctgtcatctgctgtcgcaggtcgtgcactgtgttgtccttgctgagcatgctcctctgcatgtcctctaccttggccataagcctctggtactgctcctcggccacctgcaagtcgttgttggacgacgccaggctggcattttttgcctccagcatgttctgcaggtcagtcatggctcgctccaggtcccagcacgactgcttcagggtgtccacctccgagctcagcgaatcctgccgctgctggctgctgtggctgcactccacctgcgcctgcagcttcgtgctgagggcggccagctgggcctgcagctcagccttctctttaagtgcctgactcgcctccagtgacaaggcttccagctgtccttcgagtcgcattttctctttgagcacctgcagcatctcctcctgtgtttctgctgcagagctctccaaggacacgctgctgcagatgctgtctctccgactccgcacctccccgttgacctcctgcccctggtcttggtgctcagcggctgcggcctggaggacgtccttaatggaggggaactggcccagggtatccgcaggaatctcctggccgttgaccatatagggggtgtcctgcgtgcccactgtcttcgacagaatgccataggtccctcgggtggaggcgctgctgtacgatgagctgtcgctgtcatttccatccacctcagacacgctgtctccagccagggaggtgttctccagacggtcgtcagtgtcgggggacaggctgatctcagacacaacggacgccgcactgcttctgttctgcttcagggaacccttggtagaatcgggagccgggacatttcccccagaattccccgcatttgaatcttcagttctgtaatcggccagagaccggattttgcttgatttggaagtttttttctccctaggatgtgccggaagccccaggctgcccaccttaggcccccgagggacactggtgcgcaggaaggaatattcttttgtcatagccagggtactggcccttggtaagttttctgggtttaacatgagctcaggatcaagcgtgctaaaaagtctcgttttggttgcaggttgactggacttaaaggtataagaagaacacgctggtcattttattgatcttcttctactgaagagatccttttgaaacatgacataggctgggcgcgatggtgggtgcctgtagtccc

SEQ ID NO: 18250 - RNA, 3346 nt, Homo sapiens
  source 1..3346: mol_type = other RNA
tgaagtaccagctactcgagaggctgaggcaggagaatcgcatgaacctgggaggcggagcttgcagtgagcggagagtgtgccactgcactccagcctgggcaacaaagcgagactctgtctcaaaaaaaaaaaaaaaaaaaaaacaaagattggattatgatattcagtatctatgtacacatcctatggtgggatggctatccaaaaaaacaagtaaaaagccaaaggtacagataaaatttcatttctgcggaaaagtaaagctcttactgaatggaacagggaagtgagaaactgcagccggcctggccaggcgcggtgccgcagaccctgtcacacagctgctcccagttacgcagcctctccctgtcacccgcagagagcagcatcggtggccgctcagaagccacgacctacaagtaacccttcagacacgttcaaagctcctcgccgagagcctatcaggcttttaagagttggtcattccatgtgaaaagctaattgtgatcttcgaatgtttttctagtccttggctctcattctgctatatattttacttcttgttaaaggcaaaacaaaacttaaatttcatgtcttagaaaaacatcgaccacacaatcaaataaataacattgataagagccttctggggcagcggcgcacggaggcgagtccacagcagtcactctcccggcccttctttggaagccctgctctgactgtgtctctgtgggtcgccgcgtgggccggcgtgaccccccgggggcacagggctggcagtggctggctccagcggcgtccacgaggacagagactcgtgcaccgtcagggcgtgctcctccatctggcgctgcaggctgtccatctcctgcttgagctgctggaggcagctgttcaggttcttgaggggctccttgctcacggcgggcggtggtctcagcagctcctccagcagcgaggcgggaactgggcagtccgggatcttgatgggcgtggcagggttggaagagctggcctcgcctttcggctcctttctcgtcttggccgcgccgcggcgtaggtccagcttgagctgctggttctgctggagcagggtcttcatgttgttcttcagctccgacacttttgcctggagcataaatttatccttctgggtcatggacaggtcttcctgggccatctccaactcagacttgacgttctgcagcagctgctgtagcccttccagttccttcctgccctgctgctccgtcaagtccagctgctgcttcaaggactggatttctctttctttctgatccacctcccatttgagattttccatctcttggtttcccacgggctgtttgctgagctgctcgtccagctgcttctgcaggagctggagctgtgcccgggcctcggccagctctgcttggaactgtgctatctcctgggaatgtttcccctcccgaatctgaaggtcgtcggcctcggcctgcagcttctgcaccaggtgttccttggcctgcagctccttcttcacctcactcagctccaaggaggccgccttgaagtggcggcggttatgcccggcttccaccttggcagcagccacctgctccttgaggctgttcaccttctccttctccttctctagtgaggcctgcagggcctggacaagatgcttcatctggcgatcctcctcttctttgcgctgcaaaactgcctgcacctgaaggttcaactggactaggtctgcctccctcttggccaaagctgtttctaggatgctgttgtgttcccgcagagctgcgttggactgaccgaggcccgtaagcttccctttctcgtgctctaattcaagagccaacttcttgtttgactcctcaaggcgttttatcttcttcctaaagcctctggattcttgaagctcgtcctccagctccagcaccttctcccgggactcctccagctcctggctggtcagcgctatgacctcctgcagttccttttccagcagcgtcttgctatgactgacagcctgcagctccgcctccagggcctggatcctttcatgtagagccaggctgctgtcactgctgccaccctgggctcggagctggcccagctccgcgtccgcagcctccttggccgcgagggcctcctgcaggcggcggctgaggatgcccacggcgttctcgtaggccttatgtttggtcttcatctccttctgggcgctggtcaagtctgagcccagccgcctcatcttctgcttctgttccgtgatggccttccgggcctcttgctgcaactcttcgatttgtttcttcagcgcctcattggcctctgtgaccgcgaccatctgctccttatcgaactgcaacgactgcaagtgtgtttccatctcgtctcgctccttctgcgccgactggagatgcccttcaaggtccgccatgtgctgacggacctgggccacctctctgtgcaggcgcgagagctccgcctcggcagtccgcttctccccgtgcacttgcatcagctcctgccgcagctccttcagctccgagtccagcctcttcctggtggctttcagctcactgatgagctggtctttggaggtggcgtcgcgccggtaggcctccaccatcaccttttgttggagaaactgttcctttattttttgcatttgctttttcagagcagcagtctcctgctgcaggtgttccacctggccggatttgatagctaattcttctcttaacttctctaaagtttccgacgtttcctcggtaccttcttccaagcgtcttgctcctctgtcaagctcctccttgccactcttggccgcctgcaaagccgcctccaagatgatcttctcgttctgcaggaggcagatcgtgtcctccctggaggcggcctcgccctgcagctcccccagcctggcctgcagctcatcgtagtgtgtctgcagggcatcgagggactgctccctgctctgcagagcctcctgagtcaaggtgagctgtttcatcaggtccaggtgctcctgctgcaaagcctcaagctgctggtctcgctggagtaaagtcaacttcacctgctccagctgctgctccagggatgccgccgagtccgccatcctctgcagccgctccctctcaccttcaaactcttccagcctcctctgaaggtcctcctccaccatcgtctttgcctcctgaatctgcatgaaggctgcttcctgatccaacatgtcagcctgagcccaggaaactcaatgccctgcagctgtgccgcgatgcgccccttctccttcatggacctgtgctgagtttccgtcagctgctgggacagggacaca

SEQ ID NO: 18251 - RNA, 5668 nt, Homo sapiens
  source 1..5668: mol_type = other RNA
tgaagtaccagctactcgagaggctgaggcaggagaatcgcctgaacatgggaggcagagattgtagtgagccaagattgcgccactgcacttcagcccgggagacagtgtgagactctgtctcgacaataagtaaattaaaagataaataaatcaaataaaatgcaccccagagggctcgctcactcttttttttttttaaaccatgtgaggatatgatgagaagttggcagtcggcaacacggaaggggaccctcaccagaacctgaccatgctggcatcctgattttaaacttttagcctccggaactgtgagaaataaatttttgttgtttataagccacccagttcatggtattttattacagcattctgagataagacagttattaaaaaattcccaggtatgctaataacagcaggccaatgggaattgagcctcatcaagacttcagacagagcctactaaaaagttgtgaagagttggatgaataagacatgaggcagagtcctcttgtaataaatagatgcacagcaaaccatggacctgacctggactctcctggggtcatctgatgcagtggtggtaggaagcctcttaaatactttctgactctccatgtttgcaaagagagttgaatgacatgttgaatcaaagcccatgcctgagatggctaataaaaagtctagaaaaggattatggtgatcaggagctctggaaaatccacagtagaaagcaaatttgaacctgttagggaaacacagtttaaacaatatcatgttccttgagaagaatgtttactaggagcctgatattacaaaggtgagatttgcttatacatgagtttcttagactgtgattcaattttggcatctaggcttaaagtaattctaggctattttcattttgatttgcattttttgtgtgttactaattaccaaactgaaaactatggcccttagagaaagaaagagaggtgttgatagatgtcttcatggaacaagataattcagatatcagagttagtgatgcaggttgagcatcccacatccaaaaagccaaaatccaaaatgctctaaaattcaaaactttttgagtgccaacatgatgctgaaaggaaatgcttactggaaaattttggattttgtgtgtaggatgatcaactggtaagtatacataatgcatatattccaaaatccaaaaacatcccccaaaatccaaaatctgaaacacttctggtcccaagcattcaggataaggatattcaacctatactgtgttttcaaaatgagaagagatgaccattcccttctccttcccttggagacttgagcaatcccataattgtggggatcataaaaggaaaactcaggagaaaaagcacaaagaaagaggagggatatttacttgccaagctttgcgggggaataggagcgtaccctagggttgggggcagtgggagaggtccaccttttgtcatcaccatagtccagcaattctaaataatgtcgatgataacacattcctgcctgctaggaaattattcctgtctctcaacccccatcccttctctacattaggcagcaactacaagggagtccagcctttggaagaacttgcttgccatataaaataatacaataggtgttaaaagaaaatgctccaagtttattaagactacaacctgtttatttacagaggtaaacatcatttttttcccccatatgattattatgtctgtgagggatatgggtcatcacatacatgtagccatcaggacagtaaaacttaagggagcttcagtaactcacaggcaagtgtttatttaggattttatctgtatcgtgaccaatgtcaaagggaagatcctttttttgtttatctcaggatgaaattctgctttcttgggagaaatgcaataccagacactggtctttactttttccttgattgattttagagtgggaggtccattcaaagataacatggtaagttggtcagcttcctttctactttggaccataacttaaaatagaccaatgaattcctatttgttcttcagaatatctggattaagtttcttgaatgatcatggatgatctgtggagatttggagcataatgtattttgttttgttttcttcttctttaatgtagtttatttgtaaagtcaaagaagctgctaatgaccagcttttcaaagatgtaatagaaacaagggaggaagactcataaaacacttgttcatcaaacactgtttgatgaacagcaacactagcagatattttaaagaaaaggctgctttctggccagccccataaagtcattggctgattttacaaatgtattcatggtgcggggaaccaagagccaggtttatgccaattgagctgtctgggaagttgagggcagctggaggtatatttaaactgtcagtgtaaaaatggctttgtcagccaagtggcattttctttcctctgttggggaggtgtggtgcagacaaagaaaaagaatatcacctgctcaagttggcatttcctgaagggaggaaaagttgctgcctctgtttagttcataaccagttggagaatgagtcagcaagagacagaaagtctttggagatgagtaatcatctttcagtgctggactgaggctgtcagggtggaaaatgaatgggtcttgtgcctaccctcaagtgacagggacccttaactgcaatttgctctgtcacaaggatgtgaaattgtgaattttagtatcatgaaaaatgagaatatttttgacacaattgtcagatcacatacagtaccaaaatgagaggagagattttcatgggactatcaggactgcagacttaataagtgactctgtaggattttaatttctgataaaagattacttttcttcttggtaatggatgcatttctaccataccttcctcgaaggaactcaaagtacttcacaggcgtgaatggagctggggggtgggttggacatcaggagtgaaggagttgcttcatacacacggatgatggtggtggcgggggacggccactaacagttactgagtctttgcaactttacaagttttgttttacttaatctttacgtgggttagttatttctatcctacatacaaggaaacaaaggctgggtggttatttaattcacttgaggtcacccagctattctgtgtctgagctggaataggaagacagttgtaaattctgggctctttctataaccacacatcgtacccacatggggtgggtttctgggaagatgagctgcccaggcacgggtggttacccacagagatggatctgggaggggattatccctcccactgctttggaaaatgctaaaatttcaagttaaaaatgtcttttgcagtacctgactctgagcttaagtcaggacactaccacggttcctgaaaaccagatagaaatgctagctctttcagaggtggacatggcggcacctagacatcaaatgcaggtgctgtatcagatgttcatggaggcaggtcccacagtggtctcactgtgcccacatgccttccctagtggggtgcccactaacttcctgaggagaagatgaagaaggccctgcaccaaaactagatcttcacatttattttaaacaaatagcaggagattacaaaacaggaagttccttgaactgttgatgggaatcgccaagcatggagaaatgcctaggagctttctcccacgttgatgtagaatgttcagttcagcttaattcaactttttgctttttcactgtgtttattattgtttcatggaaggcaaaatccatgtagaaaagattgaagtttgtaaatttctcactggctgcaatttttttcagtgtgttggagagttgctctgctctctctgaagtgagagtccgcaacgtcttgttggaagacatccagccgtggcaggggctgacctggaggcagttcaggaaggagtacaactgcgcataggtcatgtctttatttagctggccgagaggatgatatctgttgtgcaaattatcccagagaaaggttccatctggtaagccatacaaaataacatggctgccattgggcaggtgggaatttagatgcttcagagtctgcatgacgttggagtagagtttctcaggagtggtcatggctgggactgggtcactcttcccactgcagacatcatttccaatcatggcatatataacgatggcgggatagtccaacaccttgtttctagacaagctttctataaatttcttcaggtttcgggaagatgcaccatttcttgaaatattctggtagtccctgtgattacagtggtttcttttccataagcgaaggtaaatagatttttctttaattccaacagtggagtccagaaatcctgtagcaccagagagttggggccagtcaagctcgttggtaagggctgttggtagattgatgaaagagttcaaagacatctgcgacgctgtgatccattcaggagagatgtgaaaatgagccccagctgagtctcccagcaaaatgattcccctgggctgtgaaccttcacagaatttcttctcatatggaactccatcttttggatcgacaccccaaatgccattacagtttgaatcctgatggacatcccagttgttcggccttctacctgggtacactgactcgtcgctgtcattacagtctctcccccgccagtgatagccccgcagtgttgggaaaacgctgtatttgtctgaatccacatctttgaatggcacagactgttccatagctaatttaattttctggcagatcttggccaaaaccgggagtgaacaaatgtcagaaccacttctagaatatttcagaatcggggacttcttgacaatttgtcttgccttctgtagtgtaaatttccatgtctccttgggaagagggtagagatgacacaatggttggccagtgttctgtttacaaaactccagagtgtgacataccacatcagcattcatatctgcgctaagcagttttatgatgtctgatccaaacttgtcaatgactaaatagcaggtggttttcaagaacagtttttcaggcaggtagctgcacagtctctccatcgaggcctggaccgtcgagttgtgaacttgagcaagctgttctattacagacaccaccagcacacaccctacacaggtgtgcccattcgagaggctgggcctggactggtcatcgttggctggagaggccgaggactgaagagacaggagcaagaatagaggcgccaccgtaaggattttccagggggactgcatctccgagctatgcaccccaagtgatcacccggctttggaagctcccaactgagggatgctggagctgaggctgcagaatcaattgatctctctctccttctcttcctcactctctttgacacacacaccccaccctctcacatacacacttttcaataagtgtgaagtgaataaaagcacacataaacactcacagacccacagcttgctcttgttggaccctgagagagccacacacaaagagctggagggagtctgtggtgtgcggttctgctgaggtaaagactgcaggataaagaaaacccaagttgcacagtggcacaacttccgtgctccctggctcagt

SEQ ID NO: 18252 - RNA, 296 nt, Homo sapiens
  source 1..296: mol_type = other RNA
tgaagtaccagctactcgagaggctgaggcaggagaatcgcttgaacccaagaggcagaggttgcggtgagccgagatcgtgccattgcactccagcctgggcaacaagagtgaaactcgggagctggctaagcgtgggagccgacgtgcgccccggcctgaggagtgggacgcggccacggcgcgcggccctacaccgggacctcgttcggcgcggcgagtcggacgctcactccagccgccgccgccgccgcggctgctgcttcgccaccttggccgccatcttgactcaaccc

SEQ ID NO: 18253 - RNA, 301 nt, Homo sapiens
  source 1..301: mol_type = other RNA
tgaagtaccagctactcgagaggctgaggcaggagaatcgcttgaacccaagaggcagaggttgcggtgagccgagatcgtgccattgcactccagcctgggcaacaagagtgaaactcgggagctggctaagcgtgggagccgacgtgcgccccggcctgaggagtgggacgcggccacggcgcgcggccctacaccgggacctcgttcggcgcggcgagtcggacgctcactccagccgccgccgccgccgcggctgctgcttcgccaccttggccgccatcttgactcaacccctctc

SEQ ID NO: 18254 - RNA, 311 nt, Homo sapiens
  source 1..311: mol_type = other RNA
tgaagtaccagctactcgagaggctgaggcaggagaatcgcttgaacccaagaggcagaggttgcggtgagccgagatcgtgccattgcactccagcctgggcaacaagagtgaaactcgggagctggctaagcgtgggagccgacgtgcgccccggcctgaggagtgggacgcggccacggcgcgcggccctacaccgggacctcgttcggcgcggcgagtcggacgctcactccagccgccgccgccgccgcggctgctgcttcgccaccttggccgccatcttgactcaacccctctccctcccccca

SEQ ID NO: 18255 - RNA, 313 nt, Homo sapiens
  source 1..313: mol_type = other RNA
tgaagtaccagctactcgagaggctgaggcaggagaatcgcttgaacccaagaggcagaggttgcggtgagccgagatcgtgccattgcactccagcctgggcaacaagagtgaaactcgggagctggctaagcgtgggagccgacgtgcgccccggcctgaggagtgggacgcggccacggcgcgcggccctacaccgggacctcgttcggcgcggcgagtcggacgctcactccagccgccgccgccgccgcggctgctgcttcgccaccttggccgccatcttgactcaacccctctccctccccccagc

SEQ ID NO: 18256 - RNA, 315 nt, Homo sapiens
  source 1..315: mol_type = other RNA
tgaagtaccagctactcgagaggctgaggcaggagaatcgcttgaacccaagaggcagaggttgcggtgagccgagatcgtgccattgcactccagcctgggcaacaagagtgaaactcgggagctggctaagcgtgggagccgacgtgcgccccggcctgaggagtgggacgcggccacggcgcgcggccctacaccgggacctcgttcggcgcggcgagtcggacgctcactccagccgccgccgccgccgcggctgctgcttcgccaccttggccgccatcttgactcaacccctctccctccccccagccc

SEQ ID NO: 18257 - RNA, 316 nt, Homo sapiens
  source 1..316: mol_type = other RNA
tgaagtaccagctactcgagaggctgaggcaggagaatcgcttgaacccaagaggcagaggttgcggtgagccgagatcgtgccattgcactccagcctgggcaacaagagtgaaactcgggagctggctaagcgtgggagccgacgtgcgccccggcctgaggagtgggacgcggccacggcgcgcggccctacaccgggacctcgttcggcgcggcgagtcggacgctcactccagccgccgccgccgccgcggctgctgcttcgccaccttggccgccatcttgactcaacccctctccctccccccagcccg

SEQ ID NO: 18258 - RNA, 317 nt, Homo sapiens
  source 1..317: mol_type = other RNA
tgaagtaccagctactcgagaggctgaggcaggagaatcgcttgaacccaagaggcagaggttgcggtgagccgagatcgtgccattgcactccagcctgggcaacaagagtgaaactcgggagctggctaagcgtgggagccgacgtgcgccccggcctgaggagtgggacgcggccacggcgcgcggccctacaccgggacctcgttcggcgcggcgagtcggacgctcactccagccgccgccgccgccgcggctgctgcttcgccaccttggccgccatcttgactcaacccctctccctccccccagcccgc

SEQ ID NO: 18259 - RNA, 320 nt, Homo sapiens
  source 1..320: mol_type = other RNA
tgaagtaccagctactcgagaggctgaggcaggagaatcgcttgaacccaagaggcagaggttgcggtgagccgagatcgtgccattgcactccagcctgggcaacaagagtgaaactcgggagctggctaagcgtgggagccgacgtgcgccccggcctgaggagtgggacgcggccacggcgcgcggccctacaccgggacctcgttcggcgcggcgagtcggacgctcactccagccgccgccgccgccgcggctgctgcttcgccaccttggccgccatcttgactcaacccctctccctccccccagcccgcgga

SEQ ID NO: 18260 - RNA, 340 nt, Homo sapiens
  source 1..340: mol_type = other RNA
tgaagtaccagctactcgagaggctgaggcaggagaatcgcttgaacccaagaggcagaggttgcggtgagccgagatcgtgccattgcactccagcctgggcaacaagagtgaaactcgggagctggctaagcgtgggagccgacgtgcgccccggcctgaggagtgggacgcggccacggcgcgcggccctacaccgggacctcgttcggcgcggcgagtcggacgctcactccagccgccgccgccgccgcggctgctgcttcgccaccttggccgccatcttgactcaacccctctccctccccccagcccgcggagccgcggctaaggcggctcc

SEQ ID NO: 18261 - RNA, 3253 nt, Homo sapiens
  source 1..3253: mol_type = other RNA
tgaagtaccagctactcgagaggctgaggcaggagaatcgcttgaacccaggaggtggaggctgcagtgagctgaggtaacaccacagcactccagcctgggtgacaaagcaagactctgtctcaaaaaaaaattacactgaaagactttatggtaagtatttaaaactaaatataccaacctgtggtatattacacattttaatatattcttccataatgcccactaagaagaaataaatgggataaatgatgaaaaaaaataaagcaaataaacacgcttttaggaatgttttcgcatgtgtacatgtcagggcacatgaaaatgattcctcattagaactctctacatcctaaaaattacaaagaccgagtttctacttcaattttttcttctgcttgaagtatatctggatcaacatgaacaaccggaggtcgcaggataacttcaggccctccaccataaatagactgcagaaaattccatgtttcttcagaaatctggccagaatctgctccttgcctaagcatcacattaccacatttagtgactgcaatcttagtattgtcaataggacctggaggatccgaataaaaatttccaattcagtttttcttcttttttcaattttctccgcctcaatttggcaagtatgacaaatgtacagatggttgacagctggtcctccaccatacctgctatataggttatcccaaatgttctgaggcagcatcaaaaccaggtcttcaatataaccagcttttcttggaggaacacctccatgaatacaaagaaagtcattatttgaaatagggccaggttcggcaaaggtcttaaatttattaagccactgtcgagaaatataaaactgaaggaggcttggttccattatgttcaataaatttgatatccttctcctctctttttgtgcctcttcgctgctcttcctatagaaaagaacgtaagcttctgcattttgtacagtagattctgaaacttcagtgacactctgatcatcaaattcataccagagattatttagattgtttcggcagtaggctatatagtgtccactacttgcagttccatgatggcaaatgactgacagaagatcatatgtcacaatttgagctggactatccttagcaagaaatggctgaagatccaagccttctagcggaaatgaaacatgggtactgattttggtggaaaacattagttcatgtctgaatcttttaaggtggatgcacaaaatctcaggaaagttttgtactttacaaaacttcactccatttctcaactttttgcatttttcacaactgtacatattgtcaccttttagttcatctctggcaaagaaggcagcaagacaatcttgcaaggttactactggaccccaaaaccagctagggacacatgagacaacaaacctcttcacatattccatgaaaaaagctatccacccttgtggagcatatgcttcgccacatgatcctgctttgactatagaagttggatgacttgatgaatgcagcttagcaaggtcttccttgccaggaattggcaaggacagatcttgaaaggtctcgagggttacagacaccctgtcacaagtcagacactgcactgaactaatgattgttccatcaaatatgtctgaaataacacttctgtatttcttgtgctgtttttttctctttggagatgcagactgagcttttttgtgtggtggtgccaatcctggccacaaattgcctgatttaggagggcttgccgataaacgtggattaacaccttcatttgatggaaggatctgtggtgtagacaggtcattcgaatggacatcagtgatatattctgaagctctgctgtgtatttgcactttgacagtttcctggttgtttaagtcgactgtttcagatatagagtctctatctttatcaaattcgccttcagaatttactttattaatcttattgcacatcttctctttttgccaatcctttgacatttctgaattgttttcatcatcctgaattaacattgttgtttcattattatcttcagaaaagcatctagagccattttcattttctgctctatcactgttgctacaagattcacaagactgaaaatctacatccgactggctcttgtcttcttccattgtctcctcagtggttatggtttgcggatcttcttctacttccatgacttgctctttcaattcttcatgaagcaaatccattaaacatcgaaggaattcttgagcatcctgctgagaatacccccgaaatgttggatttacagttttaattccttgaaacagagtagtaggcacaacagatcctggcctgcttttatgccacagctctgtcattagtttgagataacttttacaaatggcaggtttcttatctgttcgagctagtcctccacaatcaagaaaaaactgtgtcaaaggtgggcaattagaaagagcctgcaaagctgcattcatgtaacaagtatttccaatatttttcaaacctgtaagacctctggccctaagttcatcttcttcatccgcttctatatccagatcatcaaatacggcaaccagaggagtttttaatgttgtattactgggtattttaaaatcctggacactgttttcttgtatttggtgaggttgtcttacatgaggcaatgaaggctgagttcctaatttcctatccaaaaatacttctttgctgcaagcataacaccatactcgaagagtggtaaggttcacagttagataatgctttgtctcctgagaatgtatggtgctgtgatctacttgtgattcaccacagccaacatatgaacatctattctccagacatgcccaaagatttggtccttggactttacaatcctgacaagtaccaagggatttttgtatcaaatcttcttttgttatttcaccaactgaatccaaatgtggacaatgatttcgaaaagctgacattttgttaggaattttttcctgtttcccaagactttcaaaatgaggtaacacctccacggcctggcccgcgggacccgccagctcgaccaacaacggcctgcagccgcacctccgcaagctcctcttttccttctcagctctcggagaggggcagtgtcgcgtcaggagggccggaaaacggccccgcagcgctgccctcggggggtccgcctcctgaactggccacttcccgcagcagccgcggctccttccggtgtctcc

SEQ ID NO: 18262 - RNA, 3432 nt, Homo sapiens
  source 1..3432: mol_type = other RNA
tgaagtaccagctactcgagaggctgaggcaggagaatcgcttgaacccaggaggtggaggctgcagtgagctgaggtaacaccacagcactccagcctgggtgacaaagcaagactctgtctcaaaaaaaaattacactgaaagactttatggtaagtatttaaaactaaatataccaacctgtggtatattacacattttaatatattcttccataatgcccactaagaagaaataaatgggataaatgatgaaaaaaaataaagcaaataaacacgcttttaggaatgttttcgcatgtgtacatgtcagggcacatgaaaatgattcctcattagaactctctacatcctaaaaattacaaagaccgagtttctacttcaattttttcttctgcttgaagtatatctggatcaacatgaacaaccggaggtcgcaggataacttcaggccctccaccataaatagactgcagaaaattccatgtttcttcagaaatctggccagaatctgctccttgcctaagcatcacattaccacatttagtgactgcaatcttagtattgtcaataggacctggaggatccgaataaaaatttccaattcagtttttcttcttttttcaattttctccgcctcaatttggcaagtatgacaaatgtacagatggttgacagctggtcctccaccatacctgctatataggttatcccaaatgttctgaggcagcatcaaaaccaggtcttcaatataaccagcttttcttggaggaacacctccatgaatacaaagaaagtcattatttgaaatagggccaggttcggcaaaggtcttaaatttattaagccactgtcgagaaatataaaactgaaggaggcttggttccattatgttcaataaatttgatatccttctcctctctttttgtgcctcttcgctgctcttcctatagaaaagaacgtaagcttctgcattttgtacagtagattctgaaacttcagtgacactctgatcatcaaattcataccagagattatttagattgtttcggcagtaggctatatagtgtccactacttgcagttccatgatggcaaatgactgacagaagatcatatgtcacaatttgagctggactatccttagcaagaaatggctgaagatccaagccttctagcggaaatgaaacatgggtactgattttggtggaaaacattagttcatgtctgaatcttttaaggtggatgcacaaaatctcaggaaagttttgtactttacaaaacttcactccatttctcaactttttgcatttttcacaactgtacatattgtcaccttttagttcatctctggcaaagaaggcagcaagacaatcttgcaaggttactactggaccccaaaaccagctagggacacatgagacaacaaacctcttcacatattccatgaaaaaagctatccacccttgtggagcatatgcttcgccacatgatcctgctttgactatagaagttggatgacttgatgaatgcagcttagcaaggtcttccttgccaggaattggcaaggacagatcttgaaaggtctcgagggttacagacaccctgtcacaagtcagacactgcactgaactaatgattgttccatcaaatatgtctgaaataacacttctgtatttcttgtgctgtttttttctctttggagatgcagactgagcttttttgtgtggtggtgccaatcctggccacaaattgcctgatttaggagggcttgccgataaacgtggattaacaccttcatttgatggaaggatctgtggtgtagacaggtcattcgaatggacatcagtgatatattctgaagctctgctgtgtatttgcactttgacagtttcctggttgtttaagtcgactgtttcagatatagagtctctatctttatcaaattcgccttcagaatttactttattaatcttattgcacatcttctctttttgccaatcctttgacatttctgaattgttttcatcatcctgaattaacattgttgtttcattattatcttcagaaaagcatctagagccattttcattttctgctctatcactgttgctacaagattcacaagactgaaaatctacatccgactggctcttgtcttcttccattgtctcctcagtggttatggtttgcggatcttcttctacttccatgacttgctctttcaattcttcatgaagcaaatccattaaacatcgaaggaattcttgagcatcctgctgagaatacccccgaaatgttggatttacagttttaattccttgaaacagagtagtaggcacaacagatcctggcctgcttttatgccacagctctgtcattagtttgagataacttttacaaatggcaggtttcttatctgttcgagctagtcctccacaatcaagaaaaaactgtgtcaaaggtgggcaattagaaagagcctgcaaagctgcattcatgtaacaagtatttccaatatttttcaaacctgtaagacctctggccctaagttcatcttcttcatccgcttctatatccagatcatcaaatacggcaaccagaggagtttttaatgttgtattactgggtattttaaaatcctggacactgttttcttgtatttggtgaggttgtcttacatgaggcaatgaaggctgagttcctaatttcctatccaaaaatacttctttgctgcaagcataacaccatactcgaagagtggtaaggttcacagttagataatgctttgtctcctgagaatgtatggtgctgtgatctacttgtgattcaccacagccaacatatgaacatctattctccagacatgcccaaagatttggtccttggactttacaatcctgacaagtaccaagggatttttgtatcaaatcttcttttgttatttcaccaactgaatccaaatgtggacaatgatttcgaaaagctgacattttgttaggaattttttcctgtttcccaagactttcaaaatgaggtaacacctttaaggttaatatcgttatgtgtgaatttgatcctgtcattacgatgttagctggttattttgctcattagttgaggcagtttcttcctaacatcgatggtctttacaatttggcatgtttttgcagtggctggtaccggttgttcctttccatgtttagtgcttccttcaggagctctccacggcctggcccgcgggacccgccagctcgaccaacaacggcctgcagccgcacctccgcaagctcctcttttccttctcagctctcggagaggggcagtgtcgcgtcaggagggccggaaaacggccccgcagcgctgccctcggggggtccgcctcctgaactggccacttcccgcagcagccgcggctccttccggtgtctcc

SEQ ID NO: 18263 - RNA, 3229 nt, Homo sapiens
  source 1..3229: mol_type = other RNA
tgaagtaccagctactcgagaggctgaggcaggagaatcgcttgaacccaggaggtggaggctgcagtgagctgaggtaacaccacagcactccagcctgggtgacaaagcaagactctgtctcaaaaaaaaattacactgaaagactttatggtaagtatttaaaactaaatataccaacctgtggtatattacacattttaatatattcttccataatgcccactaagaagaaataaatgggataaatgatgaaaaaaaataaagcaaataaacacgcttttaggaatgttttcgcatgtgtacatgtcagggcacatgaaaatgattcctcattagaactctctacatcctaaaaattacaaagaccgagtttctacttcaattttttcttctgcttgaagtatatctggatcaacatgaacaaccggaggtcgcaggataacttcaggccctccaccataaatagactgcagaaaattccatgtttcttcagaaatctggccagaatctgctccttgcctaagcatcacattaccacatttagtgactgcaatcttagtattgtcaataggacctggaggatccgaataaaaatttccaattcagtttttcttcttttttcaattttctccgcctcaatttggcaagtatgacaaatgtacagatggttgacagctggtcctccaccatacctgctatataggttatcccaaatgttctgaggcagcatcaaaaccaggtcttcaatataaccagcttttcttggaggaacacctccatgaatacaaagaaagtcattatttgaaatagggccaggttcggcaaaggtcttaaatttattaagccactgtcgagaaatataaaactgaaggaggcttggttccattatgttcaataaatttgatatccttctcctctctttttgtgcctcttcgctgctcttcctatagaaaagaacgtaagcttctgcattttgtacagtagattctgaaacttcagtgacactctgatcatcaaattcataccagagattatttagattgtttcggcagtaggctatatagtgtccactacttgcagttccatgatggcaaatgactgacagaagatcatatgtcacaatttgagctggactatccttagcaagaaatggctgaagatccaagccttctagcggaaatgaaacatgggtactgattttggtggaaaacattagttcatgtctgaatcttttaaggtggatgcacaaaatctcaggaaagttttgtactttacaaaacttcactccatttctcaactttttgcatttttcacaactgtacatattgtcaccttttagttcatctctggcaaagaaggcagcaagacaatcttgcaaggttactactggaccccaaaaccagctcttcacatattccatgaaaaaagctatccacccttgtggagcatatgcttcgccacatgatcctgctttgactatagaagttggatgacttgatgaatgcagcttagcaaggtcttccttgccaggaattggcaaggacagatcttgaaaggtctcgagggttacagacaccctgtcacaagtcagacactgcactgaactaatgattgttccatcaaatatgtctgaaataacacttctgtatttcttgtgctgtttttttctctttggagatgcagactgagcttttttgtgtggtggtgccaatcctggccacaaattgcctgatttaggagggcttgccgataaacgtggattaacaccttcatttgatggaaggatctgtggtgtagacaggtcattcgaatggacatcagtgatatattctgaagctctgctgtgtatttgcactttgacagtttcctggttgtttaagtcgactgtttcagatatagagtctctatctttatcaaattcgccttcagaatttactttattaatcttattgcacatcttctctttttgccaatcctttgacatttctgaattgttttcatcatcctgaattaacattgttgtttcattattatcttcagaaaagcatctagagccattttcattttctgctctatcactgttgctacaagattcacaagactgaaaatctacatccgactggctcttgtcttcttccattgtctcctcagtggttatggtttgcggatcttcttctacttccatgacttgctctttcaattcttcatgaagcaaatccattaaacatcgaaggaattcttgagcatcctgctgagaatacccccgaaatgttggatttacagttttaattccttgaaacagagtagtaggcacaacagatcctggcctgcttttatgccacagctctgtcattagtttgagataacttttacaaatggcaggtttcttatctgttcgagctagtcctccacaatcaagaaaaaactgtgtcaaaggtgggcaattagaaagagcctgcaaagctgcattcatgtaacaagtatttccaatatttttcaaacctgtaagacctctggccctaagttcatcttcttcatccgcttctatatccagatcatcaaatacggcaaccagaggagtttttaatgttgtattactgggtattttaaaatcctggacactgttttcttgtatttggtgaggttgtcttacatgaggcaatgaaggctgagttcctaatttcctatccaaaaatacttctttgctgcaagcataacaccatactcgaagagtggtaaggttcacagttagataatgctttgtctcctgagaatgtatggtgctgtgatctacttgtgattcaccacagccaacatatgaacatctattctccagacatgcccaaagatttggtccttggactttacaatcctgacaagtaccaagggatttttgtatcaaatcttcttttgttatttcaccaactgaatccaaatgtggacaatgatttcgaaaagctgacattttgttaggaattttttcctgtttcccaagactttcaaaatgaggtaacacctccacggcctggcccgcgggacccgccagctcgaccaacaacggcctgcagccgcacctccgcaagctcctcttttccttctcagctctcggagaggggcagtgtcgcgtcaggagggccggaaaacggccccgcagcgctgccctcggggggtccgcctcctgaactggccacttcccgcagcagccgcggctccttccggtgtctcc

SEQ ID NO: 18264 - RNA, 2810 nt, Homo sapiens
  source 1..2810: mol_type = other RNA
tgaagtaccagctactcgagaggctgaggcaggagaatcgcttgaacccaggaggtggaggctgcagtgagctgaggtaacaccacagcactccagcctgggtgacaaagcaagactctgtctcaaaaaaaaattacactgaaagactttatggtaagtatttaaaactaaatataccaacctgtggtatattacacattttaatatattcttccataatgcccactaagaagaaataaatgggataaatgatgaaaaaaaataaagcaaataaacacgcttttaggaatgttttcgcatgtgtacatgtcagggcacatgaaaatgattcctcattagaactctctacatcctaaaaattacaaagaccgagtttctacttcaattttttcttctgcttgaagtatatctggatcaacatgaacaaccggaggtcgcaggataacttcaggccctccaccataaatagactgcagaaaattccatgtttcttcagaaatctggccagaatctgctccttgcctaagcatcacattaccacatttagtgactgcaatcttagtattgtcaataggacctggaggatccgaataaaaatttccaattcagtttttcttcttttttcaattttctccgcctcaatttggcaagtatgacaaatgtacagatggttgacagctggtcctccaccatacctgctatataggttatcccaaatgttctgaggcagcatcaaaaccaggtcttcaatataaccagcttttcttggaggaacactacttgcagttccatgatggcaaatgactgacagaagatcatatgtcacaatttgagctggactatccttagcaagaaatggctgaagatccaagccttctagcggaaatgaaacatgggtactgattttggtggaaaacattagttcatgtctgaatcttttaaggtggatgcacaaaatctcaggaaagttttgtactttacaaaacttcactccatttctcaactttttgcatttttcacaactgtacatattgtcaccttttagttcatctctggcaaagaaggcagcaagacaatcttgcaaggttactactggaccccaaaaccagctagggacacatgagacaacaaacctcttcacatattccatgaaaaaagctatccacccttgtggagcatatgcttcgccacatgatcctgctttgactatagaagttggatgacttgatgaatgcagcttagcaaggtcttccttgccaggaattggcaaggacagatcttgaaaggtctcgagggttacagacaccctgtcacaagtcagacactgcactgaactaatgattgttccatcaaatatgtctgaaataacacttctgtatttcttgtgctgtttttttctctttggagatgcagactgagcttttttgtgtggtggtgccaatcctggccacaaattgcctgatttaggagggcttgccgataaacgtggattaacaccttcatttgatggaaggatctgtggtgtagacaggtcattcgaatggacatcagtgatatattctgaagctctgctgtgtatttgcactttgacagtttcctggttgtttaagtcgactgtttcagatatagagtctctatctttatcaaattcgccttcagaatttactttattaatcttattgcacatcttctctttttgccaatcctttgacatttctgaattgttttcatcatcctgaattaacattgttgtttcattattatcttcagaaaagcatctagagccattttcattttctgctctatcactgttgctacaagattcacaagactgaaaatctacatccgactggctcttgtcttcttccattgtctcctcagtggttatggtttgcggatcttcttctacttccatgacttgctctttcaattcttcatgaagcaaatccattaaacatcgaaggaattcttgagcatcctgctgagaatacccccgaaatgttggatttacagttttaattccttgaaacagagtagtaggcacaacagatcctggcctgcttttatgccacagctctgtcattagtttgagataacttttacaaatggcaggtttcttatctgttcgagctagtcctccacaatcaagaaaaaactgtgtcaaaggtgggcaattagaaagagcctgcaaagctgcattcatgtaacaagtatttccaatatttttcaaacctgtaagacctctggccctaagttcatcttcttcatccgcttctatatccagatcatcaaatacggcaaccagaggagtttttaatgttgtattactgggtattttaaaatcctggacactgttttcttgtatttggtgaggttgtcttacatgaggcaatgaaggctgagttcctaatttcctatccaaaaatacttctttgctgcaagcataacaccatactcgaagagtggtaaggttcacagttagataatgctttgtctcctgagaatgtatggtgctgtgatctacttgtgattcaccacagccaacatatgaacatctattctccagacatgcccaaagatttggtccttggactttacaatcctgacaagtaccaagggatttttgtatcaaatcttcttttgttatttcaccaactgaatccaaatgtggacaatgatttcgaaaagctgacattttgttaggaattttttcctgtttcccaagactttcaaaatgaggtaacacctttaaggttaatatcgttatgtgtgaatttgatcctgtcattacgatgttagctggttatttt

SEQ ID NO: 18265 - RNA, 3356 nt, Homo sapiens
  source 1..3356: mol_type = other RNA
tgaagtaccagctactcgagaggctgaggcaggagaatcgcttgaacccaggaggtggaggctgcagtgagctgaggtaacaccacagcactccagcctgggtgacaaagcaagactctgtctcaaaaaaaaattacactgaaagactttatggtaagtatttaaaactaaatataccaacctgtggtatattacacattttaatatattcttccataatgcccactaagaagaaataaatgggataaatgatgaaaaaaaataaagcaaataaacacgcttttaggaatgttttcgcatgtgtacatgtcagggcacatgaaaatgattcctcattagaactctctacatcctaaaaattacaaagaccgagtttctacttcaattttttcttctgcttgaagtatatctggatcaacatgaacaaccggaggtcgcaggataacttcaggccctccaccataaatagactgcagaaaattccatgtttcttcagaaatctggccagaatctgctccttgcctaagcatcacattaccacatttagtgactgcaatcttagtattgtcaataggacctggaggatctccatctttacccttcacaaaactttcccattctctaaaccactgcatactgatgcaataaaaagtagctggagagtcctctttttggaacgctctgttaagccgaataaaaatttccaattcagtttttcttcttttttcaattttctccgcctcaatttggcaagtatgacaaatgtacagatggttgacagctggtcctccaccatacctgctatataggttatcccaaatgttctgaggcagcatcaaaaccaggtcttcaatataaccagcttttcttggaggaacacctccatgaatacaaagaaagtcattatttgaaatagggccaggttcggcaaaggtcttaaatttattaagccactgtcgagaaatataaaactgaaggaggcttggttccattatgttcaataaatttgatatccttctcctctctttttgtgcctcttcgctgctcttcctatagaaaagaacgtaagcttctgcattttgtacagtagattctgaaacttcagtgacactctgatcatcaaattcataccagagattatttagattgtttcggcagtaggctatatagtgtccactacttgcagttccatgatggcaaatgactgacagaagatcatatgtcacaatttgagctggactatccttagcaagaaatggctgaagatccaagccttctagcggaaatgaaacatgggtactgattttggtggaaaacattagttcatgtctgaatcttttaaggtggatgcacaaaatctcaggaaagttttgtactttacaaaacttcactccatttctcaactttttgcatttttcacaactgtacatattgtcaccttttagttcatctctggcaaagaaggcagcaagacaatcttgcaaggttactactggaccccaaaaccagctagggacacatgagacaacaaacctcttcacatattccatgaaaaaagctatccacccttgtggagcatatgcttcgccacatgatcctgctttgactatagaagttggatgacttgatgaatgcagcttagcaaggtcttccttgccaggaattggcaaggacagatcttgaaaggtctcgagggttacagacaccctgtcacaagtcagacactgcactgaactaatgattgttccatcaaatatgtctgaaataacacttctgtatttcttgtgctgtttttttctctttggagatgcagactgagcttttttgtgtggtggtgccaatcctggccacaaattgcctgatttaggagggcttgccgataaacgtggattaacaccttcatttgatggaaggatctgtggtgtagacaggtcattcgaatggacatcagtgatatattctgaagctctgctgtgtatttgcactttgacagtttcctggttgtttaagtcgactgtttcagatatagagtctctatctttatcaaattcgccttcagaatttactttattaatcttattgcacatcttctctttttgccaatcctttgacatttctgaattgttttcatcatcctgaattaacattgttgtttcattattatcttcagaaaagcatctagagccattttcattttctgctctatcactgttgctacaagattcacaagactgaaaatctacatccgactggctcttgtcttcttccattgtctcctcagtggttatggtttgcggatcttcttctacttccatgacttgctctttcaattcttcatgaagcaaatccattaaacatcgaaggaattcttgagcatcctgctgagaatacccccgaaatgttggatttacagttttaattccttgaaacagagtagtaggcacaacagatcctggcctgcttttatgccacagctctgtcattagtttgagataacttttacaaatggcaggtttcttatctgttcgagctagtcctccacaatcaagaaaaaactgtgtcaaaggtgggcaattagaaagagcctgcaaagctgcattcatgtaacaagtatttccaatatttttcaaacctgtaagacctctggccctaagttcatcttcttcatccgcttctatatccagatcatcaaatacggcaaccagaggagtttttaatgttgtattactgggtattttaaaatcctggacactgttttcttgtatttggtgaggttgtcttacatgaggcaatgaaggctgagttcctaatttcctatccaaaaatacttctttgctgcaagcataacaccatactcgaagagtggtaaggttcacagttagataatgctttgtctcctgagaatgtatggtgctgtgatctacttgtgattcaccacagccaacatatgaacatctattctccagacatgcccaaagatttggtccttggactttacaatcctgacaagtaccaagggatttttgtatcaaatcttcttttgttatttcaccaactgaatccaaatgtggacaatgatttcgaaaagctgacattttgttaggaattttttcctgtttcccaagactttcaaaatgaggtaacacctccacggcctggcccgcgggacccgccagctcgaccaacaacggcctgcagccgcacctccgcaagctcctcttttccttctcagctctcggagaggggcagtgtcgcgtcaggagggccggaaaacggccccgcagcgctgccctcggggggtccgcctcctgaactggccacttcccgcagcagccgcggctccttccggtgtctcc

SEQ ID NO: 18266 - RNA, 3535 nt, Homo sapiens
  source 1..3535: mol_type = other RNA
tgaagtaccagctactcgagaggctgaggcaggagaatcgcttgaacccaggaggtggaggctgcagtgagctgaggtaacaccacagcactccagcctgggtgacaaagcaagactctgtctcaaaaaaaaattacactgaaagactttatggtaagtatttaaaactaaatataccaacctgtggtatattacacattttaatatattcttccataatgcccactaagaagaaataaatgggataaatgatgaaaaaaaataaagcaaataaacacgcttttaggaatgttttcgcatgtgtacatgtcagggcacatgaaaatgattcctcattagaactctctacatcctaaaaattacaaagaccgagtttctacttcaattttttcttctgcttgaagtatatctggatcaacatgaacaaccggaggtcgcaggataacttcaggccctccaccataaatagactgcagaaaattccatgtttcttcagaaatctggccagaatctgctccttgcctaagcatcacattaccacatttagtgactgcaatcttagtattgtcaataggacctggaggatctccatctttacccttcacaaaactttcccattctctaaaccactgcatactgatgcaataaaaagtagctggagagtcctctttttggaacgctctgttaagccgaataaaaatttccaattcagtttttcttcttttttcaattttctccgcctcaatttggcaagtatgacaaatgtacagatggttgacagctggtcctccaccatacctgctatataggttatcccaaatgttctgaggcagcatcaaaaccaggtcttcaatataaccagcttttcttggaggaacacctccatgaatacaaagaaagtcattatttgaaatagggccaggttcggcaaaggtcttaaatttattaagccactgtcgagaaatataaaactgaaggaggcttggttccattatgttcaataaatttgatatccttctcctctctttttgtgcctcttcgctgctcttcctatagaaaagaacgtaagcttctgcattttgtacagtagattctgaaacttcagtgacactctgatcatcaaattcataccagagattatttagattgtttcggcagtaggctatatagtgtccactacttgcagttccatgatggcaaatgactgacagaagatcatatgtcacaatttgagctggactatccttagcaagaaatggctgaagatccaagccttctagcggaaatgaaacatgggtactgattttggtggaaaacattagttcatgtctgaatcttttaaggtggatgcacaaaatctcaggaaagttttgtactttacaaaacttcactccatttctcaactttttgcatttttcacaactgtacatattgtcaccttttagttcatctctggcaaagaaggcagcaagacaatcttgcaaggttactactggaccccaaaaccagctagggacacatgagacaacaaacctcttcacatattccatgaaaaaagctatccacccttgtggagcatatgcttcgccacatgatcctgctttgactatagaagttggatgacttgatgaatgcagcttagcaaggtcttccttgccaggaattggcaaggacagatcttgaaaggtctcgagggttacagacaccctgtcacaagtcagacactgcactgaactaatgattgttccatcaaatatgtctgaaataacacttctgtatttcttgtgctgtttttttctctttggagatgcagactgagcttttttgtgtggtggtgccaatcctggccacaaattgcctgatttaggagggcttgccgataaacgtggattaacaccttcatttgatggaaggatctgtggtgtagacaggtcattcgaatggacatcagtgatatattctgaagctctgctgtgtatttgcactttgacagtttcctggttgtttaagtcgactgtttcagatatagagtctctatctttatcaaattcgccttcagaatttactttattaatcttattgcacatcttctctttttgccaatcctttgacatttctgaattgttttcatcatcctgaattaacattgttgtttcattattatcttcagaaaagcatctagagccattttcattttctgctctatcactgttgctacaagattcacaagactgaaaatctacatccgactggctcttgtcttcttccattgtctcctcagtggttatggtttgcggatcttcttctacttccatgacttgctctttcaattcttcatgaagcaaatccattaaacatcgaaggaattcttgagcatcctgctgagaatacccccgaaatgttggatttacagttttaattccttgaaacagagtagtaggcacaacagatcctggcctgcttttatgccacagctctgtcattagtttgagataacttttacaaatggcaggtttcttatctgttcgagctagtcctccacaatcaagaaaaaactgtgtcaaaggtgggcaattagaaagagcctgcaaagctgcattcatgtaacaagtatttccaatatttttcaaacctgtaagacctctggccctaagttcatcttcttcatccgcttctatatccagatcatcaaatacggcaaccagaggagtttttaatgttgtattactgggtattttaaaatcctggacactgttttcttgtatttggtgaggttgtcttacatgaggcaatgaaggctgagttcctaatttcctatccaaaaatacttctttgctgcaagcataacaccatactcgaagagtggtaaggttcacagttagataatgctttgtctcctgagaatgtatggtgctgtgatctacttgtgattcaccacagccaacatatgaacatctattctccagacatgcccaaagatttggtccttggactttacaatcctgacaagtaccaagggatttttgtatcaaatcttcttttgttatttcaccaactgaatccaaatgtggacaatgatttcgaaaagctgacattttgttaggaattttttcctgtttcccaagactttcaaaatgaggtaacacctttaaggttaatatcgttatgtgtgaatttgatcctgtcattacgatgttagctggttattttgctcattagttgaggcagtttcttcctaacatcgatggtctttacaatttggcatgtttttgcagtggctggtaccggttgttcctttccatgtttagtgcttccttcaggagctctccacggcctggcccgcgggacccgccagctcgaccaacaacggcctgcagccgcacctccgcaagctcctcttttccttctcagctctcggagaggggcagtgtcgcgtcaggagggccggaaaacggccccgcagcgctgccctcggggggtccgcctcctgaactggccacttcccgcagcagccgcggctccttccggtgtctcc

SEQ ID NO: 18267 - RNA, 3408 nt, Homo sapiens
  source 1..3408: mol_type = other RNA
tgaagtaccagctactcgagaggctgaggcaggagaatcgcttgaacccaggaggtggaggctgcagtgagctgaggtaacaccacagcactccagcctgggtgacaaagcaagactctgtctcaaaaaaaaattacactgaaagactttatggtaagtatttaaaactaaatataccaacctgtggtatattacacattttaatatattcttccataatgcccactaagaagaaataaatgggataaatgatgaaaaaaaataaagcaaataaacacgcttttaggaatgttttcgcatgtgtacatgtcagggcacatgaaaatgattcctcattagaactctctacatcctaaaaattacaaagaccgagtttctacttcaattttttcttctgcttgaagtatatctggatcaacatgaacaaccggaggtcgcaggataacttcaggccctccaccataaatagactgcagaaaattccatgtttcttcagaaatctggccagaatctgctccttgcctaagcatcacattaccacatttagtgactgcaatcttagtattgtcaataggacctggaggatctccatctttacccttcacaaaactttcccattctctaaaccactgcatactgatgcaataaaaagtagctggagagtcctctttttggaacgctctgttaagccgaataaaaatttccaattcagtttttcttcttttttcaattttctccgcctcaatttggcaagtatgacaaatgtacagatggttgacagctggtcctccaccatacctgctatataggttatcccaaatgttctgaggcagcatcaaaaccaggtcttcaatataaccagcttttcttggaggaacacctccatgaatacaaagaaagtcattatttgaaatagggccaggttcggcaaaggtcttaaatttattaagccactgtcgagaaatataaaactgaaggaggcttggttccattatgttcaataaatttgatatccttctcctctctttttgtgcctcttcgctgctcttcctatagaaaagaacgtaagcttctgcattttgtacagtagattctgaaacttcagtgacactctgatcatcaaattcataccagagattatttagattgtttcggcagtaggctatatagtgtccactacttgcagttccatgatggcaaatgactgacagaagatcatatgtcacaatttgagctggactatccttagcaagaaatggctgaagatccaagccttctagcggaaatgaaacatgggtactgattttggtggaaaacattagttcatgtctgaatcttttaaggtggatgcacaaaatctcaggaaagttttgtactttacaaaacttcactccatttctcaactttttgcatttttcacaactgtacatattgtcaccttttagttcatctctggcaaagaaggcagcaagacaatcttgcaaggttactactggaccccaaaaccagctagggacacatgagacaacaaacctcttcacatattccatgaaaaaagctatccacccttgtggagcatatgcttcgccacatgatcctgctttgactatagaagttggatgacttgatgaatgcagcttagcaaggtcttccttgccaggaattggcaaggacagatcttgaaaggtctcgagggttacagacaccctgtcacaagtcagacactgcactgaactaatgattgttccatcaaatatgtctgaaataacacttctgtatttcttgtgctgtttttttctctttggagatgcagactgagcttttttgtgtggtggtgccaatcctggccacaaattgcctgatttaggagggcttgccgataaacgtggattaacaccttcatttgatggaaggatctgtggtgtagacaggtcattcgaatggacatcagtgatatattctgaagctctgctgtgtatttgcactttgacagtttcctggttgtttaagtcgactgtttcagatatagagtctctatctttatcaaattcgccttcagaatttactttattaatcttattgcacatcttctctttttgccaatcctttgacatttctgaattgttttcatcatcctgaattaacattgttgtttcattattatcttcagaaaagcatctagagccattttcattttctgctctatcactgttgctacaagattcacaagactgaaaatctacatccgactggctcttgtcttcttccattgtctcctcagtggttatggtttgcggatcttcttctacttccatgacttgctctttcaattcttcatgaagcaaatccattaaacatcgaaggaattcttgagcatcctgctgagaatacccccgaaatgttggatttacagttttaattccttgaaacagagtagtaggcacaacagatcctggcctgcttttatgccacagctctgtcattagtttgagataacttttacaaatggcaggtttcttatctgttcgagctagtcctccacaatcaagaaaaaactgtgtcaaaggtgggtagctggttatatcggcaaagttatttaaacttctgtgtctggttttcttatcaattagaaagagcctgcaaagctgcattcatgtaacaagtatttccaatatttttcaaacctgtaagacctctggccctaagttcatcttcttcatccgcttctatatccagatcatcaaatacggcaaccagaggagtttttaatgttgtattactgggtattttaaaatcctggacactgttttcttgtatttggtgaggttgtcttacatgaggcaatgaaggctgagttcctaatttcctatccaaaaatacttctttgctgcaagcataacaccatactcgaagagtggtaaggttcacagttagataatgctttgtctcctgagaatgtatggtgctgtgatctacttgtgattcaccacagccaacatatgaacatctattctccagacatgcccaaagatttggtccttggactttacaatcctgacaagtaccaagggatttttgtatcaaatcttcttttgttatttcaccaactgaatccaaatgtggacaatgatttcgaaaagctgacattttgttaggaattttttcctgtttcccaagactttcaaaatgaggtaacacctccacggcctggcccgcgggacccgccagctcgaccaacaacggcctgcagccgcacctccgcaagctcctcttttccttctcagctctcggagaggggcagtgtcgcgtcaggagggccggaaaacggccccgcagcgctgccctcggggggtccgcctcctgaactggccacttcccgcagcagccgcggctccttccggtgtctcc

SEQ ID NO: 18268 - RNA, 3587 nt, Homo sapiens
  source 1..3587: mol_type = other RNA
tgaagtaccagctactcgagaggctgaggcaggagaatcgcttgaacccaggaggtggaggctgcagtgagctgaggtaacaccacagcactccagcctgggtgacaaagcaagactctgtctcaaaaaaaaattacactgaaagactttatggtaagtatttaaaactaaatataccaacctgtggtatattacacattttaatatattcttccataatgcccactaagaagaaataaatgggataaatgatgaaaaaaaataaagcaaataaacacgcttttaggaatgttttcgcatgtgtacatgtcagggcacatgaaaatgattcctcattagaactctctacatcctaaaaattacaaagaccgagtttctacttcaattttttcttctgcttgaagtatatctggatcaacatgaacaaccggaggtcgcaggataacttcaggccctccaccataaatagactgcagaaaattccatgtttcttcagaaatctggccagaatctgctccttgcctaagcatcacattaccacatttagtgactgcaatcttagtattgtcaataggacctggaggatctccatctttacccttcacaaaactttcccattctctaaaccactgcatactgatgcaataaaaagtagctggagagtcctctttttggaacgctctgttaagccgaataaaaatttccaattcagtttttcttcttttttcaattttctccgcctcaatttggcaagtatgacaaatgtacagatggttgacagctggtcctccaccatacctgctatataggttatcccaaatgttctgaggcagcatcaaaaccaggtcttcaatataaccagcttttcttggaggaacacctccatgaatacaaagaaagtcattatttgaaatagggccaggttcggcaaaggtcttaaatttattaagccactgtcgagaaatataaaactgaaggaggcttggttccattatgttcaataaatttgatatccttctcctctctttttgtgcctcttcgctgctcttcctatagaaaagaacgtaagcttctgcattttgtacagtagattctgaaacttcagtgacactctgatcatcaaattcataccagagattatttagattgtttcggcagtaggctatatagtgtccactacttgcagttccatgatggcaaatgactgacagaagatcatatgtcacaatttgagctggactatccttagcaagaaatggctgaagatccaagccttctagcggaaatgaaacatgggtactgattttggtggaaaacattagttcatgtctgaatcttttaaggtggatgcacaaaatctcaggaaagttttgtactttacaaaacttcactccatttctcaactttttgcatttttcacaactgtacatattgtcaccttttagttcatctctggcaaagaaggcagcaagacaatcttgcaaggttactactggaccccaaaaccagctagggacacatgagacaacaaacctcttcacatattccatgaaaaaagctatccacccttgtggagcatatgcttcgccacatgatcctgctttgactatagaagttggatgacttgatgaatgcagcttagcaaggtcttccttgccaggaattggcaaggacagatcttgaaaggtctcgagggttacagacaccctgtcacaagtcagacactgcactgaactaatgattgttccatcaaatatgtctgaaataacacttctgtatttcttgtgctgtttttttctctttggagatgcagactgagcttttttgtgtggtggtgccaatcctggccacaaattgcctgatttaggagggcttgccgataaacgtggattaacaccttcatttgatggaaggatctgtggtgtagacaggtcattcgaatggacatcagtgatatattctgaagctctgctgtgtatttgcactttgacagtttcctggttgtttaagtcgactgtttcagatatagagtctctatctttatcaaattcgccttcagaatttactttattaatcttattgcacatcttctctttttgccaatcctttgacatttctgaattgttttcatcatcctgaattaacattgttgtttcattattatcttcagaaaagcatctagagccattttcattttctgctctatcactgttgctacaagattcacaagactgaaaatctacatccgactggctcttgtcttcttccattgtctcctcagtggttatggtttgcggatcttcttctacttccatgacttgctctttcaattcttcatgaagcaaatccattaaacatcgaaggaattcttgagcatcctgctgagaatacccccgaaatgttggatttacagttttaattccttgaaacagagtagtaggcacaacagatcctggcctgcttttatgccacagctctgtcattagtttgagataacttttacaaatggcaggtttcttatctgttcgagctagtcctccacaatcaagaaaaaactgtgtcaaaggtgggtagctggttatatcggcaaagttatttaaacttctgtgtctggttttcttatcaattagaaagagcctgcaaagctgcattcatgtaacaagtatttccaatatttttcaaacctgtaagacctctggccctaagttcatcttcttcatccgcttctatatccagatcatcaaatacggcaaccagaggagtttttaatgttgtattactgggtattttaaaatcctggacactgttttcttgtatttggtgaggttgtcttacatgaggcaatgaaggctgagttcctaatttcctatccaaaaatacttctttgctgcaagcataacaccatactcgaagagtggtaaggttcacagttagataatgctttgtctcctgagaatgtatggtgctgtgatctacttgtgattcaccacagccaacatatgaacatctattctccagacatgcccaaagatttggtccttggactttacaatcctgacaagtaccaagggatttttgtatcaaatcttcttttgttatttcaccaactgaatccaaatgtggacaatgatttcgaaaagctgacattttgttaggaattttttcctgtttcccaagactttcaaaatgaggtaacacctttaaggttaatatcgttatgtgtgaatttgatcctgtcattacgatgttagctggttattttgctcattagttgaggcagtttcttcctaacatcgatggtctttacaatttggcatgtttttgcagtggctggtaccggttgttcctttccatgtttagtgcttccttcaggagctctccacggcctggcccgcgggacccgccagctcgaccaacaacggcctgcagccgcacctccgcaagctcctcttttccttctcagctctcggagaggggcagtgtcgcgtcaggagggccggaaaacggccccgcagcgctgccctcggggggtccgcctcctgaactggccacttcccgcagcagccgcggctccttccggtgtctcc

SEQ ID NO: 18269 - RNA, 3332 nt, Homo sapiens
  source 1..3332: mol_type = other RNA
tgaagtaccagctactcgagaggctgaggcaggagaatcgcttgaacccaggaggtggaggctgcagtgagctgaggtaacaccacagcactccagcctgggtgacaaagcaagactctgtctcaaaaaaaaattacactgaaagactttatggtaagtatttaaaactaaatataccaacctgtggtatattacacattttaatatattcttccataatgcccactaagaagaaataaatgggataaatgatgaaaaaaaataaagcaaataaacacgcttttaggaatgttttcgcatgtgtacatgtcagggcacatgaaaatgattcctcattagaactctctacatcctaaaaattacaaagaccgagtttctacttcaattttttcttctgcttgaagtatatctggatcaacatgaacaaccggaggtcgcaggataacttcaggccctccaccataaatagactgcagaaaattccatgtttcttcagaaatctggccagaatctgctccttgcctaagcatcacattaccacatttagtgactgcaatcttagtattgtcaataggacctggaggatctccatctttacccttcacaaaactttcccattctctaaaccactgcatactgatgcaataaaaagtagctggagagtcctctttttggaacgctctgttaagccgaataaaaatttccaattcagtttttcttcttttttcaattttctccgcctcaatttggcaagtatgacaaatgtacagatggttgacagctggtcctccaccatacctgctatataggttatcccaaatgttctgaggcagcatcaaaaccaggtcttcaatataaccagcttttcttggaggaacacctccatgaatacaaagaaagtcattatttgaaatagggccaggttcggcaaaggtcttaaatttattaagccactgtcgagaaatataaaactgaaggaggcttggttccattatgttcaataaatttgatatccttctcctctctttttgtgcctcttcgctgctcttcctatagaaaagaacgtaagcttctgcattttgtacagtagattctgaaacttcagtgacactctgatcatcaaattcataccagagattatttagattgtttcggcagtaggctatatagtgtccactacttgcagttccatgatggcaaatgactgacagaagatcatatgtcacaatttgagctggactatccttagcaagaaatggctgaagatccaagccttctagcggaaatgaaacatgggtactgattttggtggaaaacattagttcatgtctgaatcttttaaggtggatgcacaaaatctcaggaaagttttgtactttacaaaacttcactccatttctcaactttttgcatttttcacaactgtacatattgtcaccttttagttcatctctggcaaagaaggcagcaagacaatcttgcaaggttactactggaccccaaaaccagctcttcacatattccatgaaaaaagctatccacccttgtggagcatatgcttcgccacatgatcctgctttgactatagaagttggatgacttgatgaatgcagcttagcaaggtcttccttgccaggaattggcaaggacagatcttgaaaggtctcgagggttacagacaccctgtcacaagtcagacactgcactgaactaatgattgttccatcaaatatgtctgaaataacacttctgtatttcttgtgctgtttttttctctttggagatgcagactgagcttttttgtgtggtggtgccaatcctggccacaaattgcctgatttaggagggcttgccgataaacgtggattaacaccttcatttgatggaaggatctgtggtgtagacaggtcattcgaatggacatcagtgatatattctgaagctctgctgtgtatttgcactttgacagtttcctggttgtttaagtcgactgtttcagatatagagtctctatctttatcaaattcgccttcagaatttactttattaatcttattgcacatcttctctttttgccaatcctttgacatttctgaattgttttcatcatcctgaattaacattgttgtttcattattatcttcagaaaagcatctagagccattttcattttctgctctatcactgttgctacaagattcacaagactgaaaatctacatccgactggctcttgtcttcttccattgtctcctcagtggttatggtttgcggatcttcttctacttccatgacttgctctttcaattcttcatgaagcaaatccattaaacatcgaaggaattcttgagcatcctgctgagaatacccccgaaatgttggatttacagttttaattccttgaaacagagtagtaggcacaacagatcctggcctgcttttatgccacagctctgtcattagtttgagataacttttacaaatggcaggtttcttatctgttcgagctagtcctccacaatcaagaaaaaactgtgtcaaaggtgggcaattagaaagagcctgcaaagctgcattcatgtaacaagtatttccaatatttttcaaacctgtaagacctctggccctaagttcatcttcttcatccgcttctatatccagatcatcaaatacggcaaccagaggagtttttaatgttgtattactgggtattttaaaatcctggacactgttttcttgtatttggtgaggttgtcttacatgaggcaatgaaggctgagttcctaatttcctatccaaaaatacttctttgctgcaagcataacaccatactcgaagagtggtaaggttcacagttagataatgctttgtctcctgagaatgtatggtgctgtgatctacttgtgattcaccacagccaacatatgaacatctattctccagacatgcccaaagatttggtccttggactttacaatcctgacaagtaccaagggatttttgtatcaaatcttcttttgttatttcaccaactgaatccaaatgtggacaatgatttcgaaaagctgacattttgttaggaattttttcctgtttcccaagactttcaaaatgaggtaacacctccacggcctggcccgcgggacccgccagctcgaccaacaacggcctgcagccgcacctccgcaagctcctcttttccttctcagctctcggagaggggcagtgtcgcgtcaggagggccggaaaacggccccgcagcgctgccctcggggggtccgcctcctgaactggccacttcccgcagcagccgcggctccttccggtgtctcc

SEQ ID NO: 18270 - RNA, 3511 nt, Homo sapiens
  source 1..3511: mol_type = other RNA
tgaagtaccagctactcgagaggctgaggcaggagaatcgcttgaacccaggaggtggaggctgcagtgagctgaggtaacaccacagcactccagcctgggtgacaaagcaagactctgtctcaaaaaaaaattacactgaaagactttatggtaagtatttaaaactaaatataccaacctgtggtatattacacattttaatatattcttccataatgcccactaagaagaaataaatgggataaatgatgaaaaaaaataaagcaaataaacacgcttttaggaatgttttcgcatgtgtacatgtcagggcacatgaaaatgattcctcattagaactctctacatcctaaaaattacaaagaccgagtttctacttcaattttttcttctgcttgaagtatatctggatcaacatgaacaaccggaggtcgcaggataacttcaggccctccaccataaatagactgcagaaaattccatgtttcttcagaaatctggccagaatctgctccttgcctaagcatcacattaccacatttagtgactgcaatcttagtattgtcaataggacctggaggatctccatctttacccttcacaaaactttcccattctctaaaccactgcatactgatgcaataaaaagtagctggagagtcctctttttggaacgctctgttaagccgaataaaaatttccaattcagtttttcttcttttttcaattttctccgcctcaatttggcaagtatgacaaatgtacagatggttgacagctggtcctccaccatacctgctatataggttatcccaaatgttctgaggcagcatcaaaaccaggtcttcaatataaccagcttttcttggaggaacacctccatgaatacaaagaaagtcattatttgaaatagggccaggttcggcaaaggtcttaaatttattaagccactgtcgagaaatataaaactgaaggaggcttggttccattatgttcaataaatttgatatccttctcctctctttttgtgcctcttcgctgctcttcctatagaaaagaacgtaagcttctgcattttgtacagtagattctgaaacttcagtgacactctgatcatcaaattcataccagagattatttagattgtttcggcagtaggctatatagtgtccactacttgcagttccatgatggcaaatgactgacagaagatcatatgtcacaatttgagctggactatccttagcaagaaatggctgaagatccaagccttctagcggaaatgaaacatgggtactgattttggtggaaaacattagttcatgtctgaatcttttaaggtggatgcacaaaatctcaggaaagttttgtactttacaaaacttcactccatttctcaactttttgcatttttcacaactgtacatattgtcaccttttagttcatctctggcaaagaaggcagcaagacaatcttgcaaggttactactggaccccaaaaccagctcttcacatattccatgaaaaaagctatccacccttgtggagcatatgcttcgccacatgatcctgctttgactatagaagttggatgacttgatgaatgcagcttagcaaggtcttccttgccaggaattggcaaggacagatcttgaaaggtctcgagggttacagacaccctgtcacaagtcagacactgcactgaactaatgattgttccatcaaatatgtctgaaataacacttctgtatttcttgtgctgtttttttctctttggagatgcagactgagcttttttgtgtggtggtgccaatcctggccacaaattgcctgatttaggagggcttgccgataaacgtggattaacaccttcatttgatggaaggatctgtggtgtagacaggtcattcgaatggacatcagtgatatattctgaagctctgctgtgtatttgcactttgacagtttcctggttgtttaagtcgactgtttcagatatagagtctctatctttatcaaattcgccttcagaatttactttattaatcttattgcacatcttctctttttgccaatcctttgacatttctgaattgttttcatcatcctgaattaacattgttgtttcattattatcttcagaaaagcatctagagccattttcattttctgctctatcactgttgctacaagattcacaagactgaaaatctacatccgactggctcttgtcttcttccattgtctcctcagtggttatggtttgcggatcttcttctacttccatgacttgctctttcaattcttcatgaagcaaatccattaaacatcgaaggaattcttgagcatcctgctgagaatacccccgaaatgttggatttacagttttaattccttgaaacagagtagtaggcacaacagatcctggcctgcttttatgccacagctctgtcattagtttgagataacttttacaaatggcaggtttcttatctgttcgagctagtcctccacaatcaagaaaaaactgtgtcaaaggtgggcaattagaaagagcctgcaaagctgcattcatgtaacaagtatttccaatatttttcaaacctgtaagacctctggccctaagttcatcttcttcatccgcttctatatccagatcatcaaatacggcaaccagaggagtttttaatgttgtattactgggtattttaaaatcctggacactgttttcttgtatttggtgaggttgtcttacatgaggcaatgaaggctgagttcctaatttcctatccaaaaatacttctttgctgcaagcataacaccatactcgaagagtggtaaggttcacagttagataatgctttgtctcctgagaatgtatggtgctgtgatctacttgtgattcaccacagccaacatatgaacatctattctccagacatgcccaaagatttggtccttggactttacaatcctgacaagtaccaagggatttttgtatcaaatcttcttttgttatttcaccaactgaatccaaatgtggacaatgatttcgaaaagctgacattttgttaggaattttttcctgtttcccaagactttcaaaatgaggtaacacctttaaggttaatatcgttatgtgtgaatttgatcctgtcattacgatgttagctggttattttgctcattagttgaggcagtttcttcctaacatcgatggtctttacaatttggcatgtttttgcagtggctggtaccggttgttcctttccatgtttagtgcttccttcaggagctctccacggcctggcccgcgggacccgccagctcgaccaacaacggcctgcagccgcacctccgcaagctcctcttttccttctcagctctcggagaggggcagtgtcgcgtcaggagggccggaaaacggccccgcagcgctgccctcggggggtccgcctcctgaactggccacttcccgcagcagccgcggctccttccggtgtctcc

SEQ ID NO: 18271 - RNA, 3059 nt, Homo sapiens
  source 1..3059: mol_type = other RNA
tgaagtaccagctactcgagaggctgaggcaggagaatcgcttgaacccaggaggtggaggctgcagtgagctgaggtaacaccacagcactccagcctgggtgacaaagcaagactctgtctcaaaaaaaaattacactgaaagactttatggtaagtatttaaaactaaatataccaacctgtggtatattacacattttaatatattcttccataatgcccactaagaagaaataaatgggataaatgatgaaaaaaaataaagcaaataaacacgcttttaggaatgttttcgcatgtgtacatgtcagggcacatgaaaatgattcctcattagaactctctacatcctaaaaattacaaagaccgagtttctacttcaattttttcttctgcttgaagtatatctggatcaacatgaacaaccggaggtcgcaggataacttcaggccctccaccataaatagactgcagaaaattccatgtttcttcagaaatctggccagaatctgctccttgcctaagcatcacattaccacatttagtgactgcaatcttagtattgtcaataggacctggaggatctccatctttacccttcacaaaactttcccattctctaaaccactgcatactgatgcaataaaaagtagctggagagtcctctttttggaacgctctgttaagccgaataaaaatttccaattcagtttttcttcttttttcaattttctccgcctcaatttggcaagtatgacaaatgtacagatggttgacagctggtcctccaccatacctgctatataggttatcccaaatgttctgaggcagcatcaaaaccaggtcttcaatataaccagcttttcttggaggaacactacttgcagttccatgatggcaaatgactgacagaagatcatatgtcacaatttgagctggactatccttagcaagaaatggctgaagatccaagccttctagcggaaatgaaacatgggtactgattttggtggaaaacattagttcatgtctgaatcttttaaggtggatgcacaaaatctcaggaaagttttgtactttacaaaacttcactccatttctcaactttttgcatttttcacaactgtacatattgtcaccttttagttcatctctggcaaagaaggcagcaagacaatcttgcaaggttactactggaccccaaaaccagctagggacacatgagacaacaaacctcttcacatattccatgaaaaaagctatccacccttgtggagcatatgcttcgccacatgatcctgctttgactatagaagttggatgacttgatgaatgcagcttagcaaggtcttccttgccaggaattggcaaggacagatcttgaaaggtctcgagggttacagacaccctgtcacaagtcagacactgcactgaactaatgattgttccatcaaatatgtctgaaataacacttctgtatttcttgtgctgtttttttctctttggagatgcagactgagcttttttgtgtggtggtgccaatcctggccacaaattgcctgatttaggagggcttgccgataaacgtggattaacaccttcatttgatggaaggatctgtggtgtagacaggtcattcgaatggacatcagtgatatattctgaagctctgctgtgtatttgcactttgacagtttcctggttgtttaagtcgactgtttcagatatagagtctctatctttatcaaattcgccttcagaatttactttattaatcttattgcacatcttctctttttgccaatcctttgacatttctgaattgttttcatcatcctgaattaacattgttgtttcattattatcttcagaaaagcatctagagccattttcattttctgctctatcactgttgctacaagattcacaagactgaaaatctacatccgactggctcttgtcttcttccattgtctcctcagtggttatggtttgcggatcttcttctacttccatgacttgctctttcaattcttcatgaagcaaatccattaaacatcgaaggaattcttgagcatcctgctgagaatacccccgaaatgttggatttacagttttaattccttgaaacagagtagtaggcacaacagatcctggcctgcttttatgccacagctctgtcattagtttgagataacttttacaaatggcaggtttcttatctgttcgagctagtcctccacaatcaagaaaaaactgtgtcaaaggtgggcaattagaaagagcctgcaaagctgcattcatgtaacaagtatttccaatatttttcaaacctgtaagacctctggccctaagttcatcttcttcatccgcttctatatccagatcatcaaatacggcaaccagaggagtttttaatgttgtattactgggtattttaaaatcctggacactgttttcttgtatttggtgaggttgtcttacatgaggcaatgaaggctgagttcctaatttcctatccaaaaatacttctttgctgcaagcataacaccatactcgaagagtggtaaggttcacagttagataatgctttgtctcctgagaatgtatggtgctgtgatctacttgtgattcaccacagccaacatatgaacatctattctccagacatgcccaaagatttggtccttggactttacaatcctgacaagtaccaagggatttttgtatcaaatcttcttttgttatttcaccaactgaatccaaatgtggacaatgatttcgaaaagctgacattttgttaggaattttttcctgtttcccaagactttcaaaatgaggtaacacctccacggcctggcccgcgggacccgccagctcgaccaacaacggcctgcagccgcacctccgcaagctcctcttttccttctcagctctcggagaggggcagtgtcgcgtcaggagggccggaaaacggccccgcagcgctgccctcggggggtccgcctcctgaactggccacttcccgcagcagccgcggctccttccggtgtctcc

SEQ ID NO: 18272 - RNA, 3238 nt, Homo sapiens
  source 1..3238: mol_type = other RNA
tgaagtaccagctactcgagaggctgaggcaggagaatcgcttgaacccaggaggtggaggctgcagtgagctgaggtaacaccacagcactccagcctgggtgacaaagcaagactctgtctcaaaaaaaaattacactgaaagactttatggtaagtatttaaaactaaatataccaacctgtggtatattacacattttaatatattcttccataatgcccactaagaagaaataaatgggataaatgatgaaaaaaaataaagcaaataaacacgcttttaggaatgttttcgcatgtgtacatgtcagggcacatgaaaatgattcctcattagaactctctacatcctaaaaattacaaagaccgagtttctacttcaattttttcttctgcttgaagtatatctggatcaacatgaacaaccggaggtcgcaggataacttcaggccctccaccataaatagactgcagaaaattccatgtttcttcagaaatctggccagaatctgctccttgcctaagcatcacattaccacatttagtgactgcaatcttagtattgtcaataggacctggaggatctccatctttacccttcacaaaactttcccattctctaaaccactgcatactgatgcaataaaaagtagctggagagtcctctttttggaacgctctgttaagccgaataaaaatttccaattcagtttttcttcttttttcaattttctccgcctcaatttggcaagtatgacaaatgtacagatggttgacagctggtcctccaccatacctgctatataggttatcccaaatgttctgaggcagcatcaaaaccaggtcttcaatataaccagcttttcttggaggaacactacttgcagttccatgatggcaaatgactgacagaagatcatatgtcacaatttgagctggactatccttagcaagaaatggctgaagatccaagccttctagcggaaatgaaacatgggtactgattttggtggaaaacattagttcatgtctgaatcttttaaggtggatgcacaaaatctcaggaaagttttgtactttacaaaacttcactccatttctcaactttttgcatttttcacaactgtacatattgtcaccttttagttcatctctggcaaagaaggcagcaagacaatcttgcaaggttactactggaccccaaaaccagctagggacacatgagacaacaaacctcttcacatattccatgaaaaaagctatccacccttgtggagcatatgcttcgccacatgatcctgctttgactatagaagttggatgacttgatgaatgcagcttagcaaggtcttccttgccaggaattggcaaggacagatcttgaaaggtctcgagggttacagacaccctgtcacaagtcagacactgcactgaactaatgattgttccatcaaatatgtctgaaataacacttctgtatttcttgtgctgtttttttctctttggagatgcagactgagcttttttgtgtggtggtgccaatcctggccacaaattgcctgatttaggagggcttgccgataaacgtggattaacaccttcatttgatggaaggatctgtggtgtagacaggtcattcgaatggacatcagtgatatattctgaagctctgctgtgtatttgcactttgacagtttcctggttgtttaagtcgactgtttcagatatagagtctctatctttatcaaattcgccttcagaatttactttattaatcttattgcacatcttctctttttgccaatcctttgacatttctgaattgttttcatcatcctgaattaacattgttgtttcattattatcttcagaaaagcatctagagccattttcattttctgctctatcactgttgctacaagattcacaagactgaaaatctacatccgactggctcttgtcttcttccattgtctcctcagtggttatggtttgcggatcttcttctacttccatgacttgctctttcaattcttcatgaagcaaatccattaaacatcgaaggaattcttgagcatcctgctgagaatacccccgaaatgttggatttacagttttaattccttgaaacagagtagtaggcacaacagatcctggcctgcttttatgccacagctctgtcattagtttgagataacttttacaaatggcaggtttcttatctgttcgagctagtcctccacaatcaagaaaaaactgtgtcaaaggtgggcaattagaaagagcctgcaaagctgcattcatgtaacaagtatttccaatatttttcaaacctgtaagacctctggccctaagttcatcttcttcatccgcttctatatccagatcatcaaatacggcaaccagaggagtttttaatgttgtattactgggtattttaaaatcctggacactgttttcttgtatttggtgaggttgtcttacatgaggcaatgaaggctgagttcctaatttcctatccaaaaatacttctttgctgcaagcataacaccatactcgaagagtggtaaggttcacagttagataatgctttgtctcctgagaatgtatggtgctgtgatctacttgtgattcaccacagccaacatatgaacatctattctccagacatgcccaaagatttggtccttggactttacaatcctgacaagtaccaagggatttttgtatcaaatcttcttttgttatttcaccaactgaatccaaatgtggacaatgatttcgaaaagctgacattttgttaggaattttttcctgtttcccaagactttcaaaatgaggtaacacctttaaggttaatatcgttatgtgtgaatttgatcctgtcattacgatgttagctggttattttgctcattagttgaggcagtttcttcctaacatcgatggtctttacaatttggcatgtttttgcagtggctggtaccggttgttcctttccatgtttagtgcttccttcaggagctctccacggcctggcccgcgggacccgccagctcgaccaacaacggcctgcagccgcacctccgcaagctcctcttttccttctcagctctcggagaggggcagtgtcgcgtcaggagggccggaaaacggccccgcagcgctgccctcggggggtccgcctcctgaactggccacttcccgcagcagccgcggctccttccggtgtctcc

SEQ ID NO: 18273 - RNA, 3035 nt, Homo sapiens
  source 1..3035: mol_type = other RNA
tgaagtaccagctactcgagaggctgaggcaggagaatcgcttgaacccaggaggtggaggctgcagtgagctgaggtaacaccacagcactccagcctgggtgacaaagcaagactctgtctcaaaaaaaaattacactgaaagactttatggtaagtatttaaaactaaatataccaacctgtggtatattacacattttaatatattcttccataatgcccactaagaagaaataaatgggataaatgatgaaaaaaaataaagcaaataaacacgcttttaggaatgttttcgcatgtgtacatgtcagggcacatgaaaatgattcctcattagaactctctacatcctaaaaattacaaagaccgagtttctacttcaattttttcttctgcttgaagtatatctggatcaacatgaacaaccggaggtcgcaggataacttcaggccctccaccataaatagactgcagaaaattccatgtttcttcagaaatctggccagaatctgctccttgcctaagcatcacattaccacatttagtgactgcaatcttagtattgtcaataggacctggaggatctccatctttacccttcacaaaactttcccattctctaaaccactgcatactgatgcaataaaaagtagctggagagtcctctttttggaacgctctgttaagccgaataaaaatttccaattcagtttttcttcttttttcaattttctccgcctcaatttggcaagtatgacaaatgtacagatggttgacagctggtcctccaccatacctgctatataggttatcccaaatgttctgaggcagcatcaaaaccaggtcttcaatataaccagcttttcttggaggaacactacttgcagttccatgatggcaaatgactgacagaagatcatatgtcacaatttgagctggactatccttagcaagaaatggctgaagatccaagccttctagcggaaatgaaacatgggtactgattttggtggaaaacattagttcatgtctgaatcttttaaggtggatgcacaaaatctcaggaaagttttgtactttacaaaacttcactccatttctcaactttttgcatttttcacaactgtacatattgtcaccttttagttcatctctggcaaagaaggcagcaagacaatcttgcaaggttactactggaccccaaaaccagctcttcacatattccatgaaaaaagctatccacccttgtggagcatatgcttcgccacatgatcctgctttgactatagaagttggatgacttgatgaatgcagcttagcaaggtcttccttgccaggaattggcaaggacagatcttgaaaggtctcgagggttacagacaccctgtcacaagtcagacactgcactgaactaatgattgttccatcaaatatgtctgaaataacacttctgtatttcttgtgctgtttttttctctttggagatgcagactgagcttttttgtgtggtggtgccaatcctggccacaaattgcctgatttaggagggcttgccgataaacgtggattaacaccttcatttgatggaaggatctgtggtgtagacaggtcattcgaatggacatcagtgatatattctgaagctctgctgtgtatttgcactttgacagtttcctggttgtttaagtcgactgtttcagatatagagtctctatctttatcaaattcgccttcagaatttactttattaatcttattgcacatcttctctttttgccaatcctttgacatttctgaattgttttcatcatcctgaattaacattgttgtttcattattatcttcagaaaagcatctagagccattttcattttctgctctatcactgttgctacaagattcacaagactgaaaatctacatccgactggctcttgtcttcttccattgtctcctcagtggttatggtttgcggatcttcttctacttccatgacttgctctttcaattcttcatgaagcaaatccattaaacatcgaaggaattcttgagcatcctgctgagaatacccccgaaatgttggatttacagttttaattccttgaaacagagtagtaggcacaacagatcctggcctgcttttatgccacagctctgtcattagtttgagataacttttacaaatggcaggtttcttatctgttcgagctagtcctccacaatcaagaaaaaactgtgtcaaaggtgggcaattagaaagagcctgcaaagctgcattcatgtaacaagtatttccaatatttttcaaacctgtaagacctctggccctaagttcatcttcttcatccgcttctatatccagatcatcaaatacggcaaccagaggagtttttaatgttgtattactgggtattttaaaatcctggacactgttttcttgtatttggtgaggttgtcttacatgaggcaatgaaggctgagttcctaatttcctatccaaaaatacttctttgctgcaagcataacaccatactcgaagagtggtaaggttcacagttagataatgctttgtctcctgagaatgtatggtgctgtgatctacttgtgattcaccacagccaacatatgaacatctattctccagacatgcccaaagatttggtccttggactttacaatcctgacaagtaccaagggatttttgtatcaaatcttcttttgttatttcaccaactgaatccaaatgtggacaatgatttcgaaaagctgacattttgttaggaattttttcctgtttcccaagactttcaaaatgaggtaacacctccacggcctggcccgcgggacccgccagctcgaccaacaacggcctgcagccgcacctccgcaagctcctcttttccttctcagctctcggagaggggcagtgtcgcgtcaggagggccggaaaacggccccgcagcgctgccctcggggggtccgcctcctgaactggccacttcccgcagcagccgcggctccttccggtgtctcc

SEQ ID NO: 18274 - RNA, 4422 nt, Homo sapiens
  source 1..4422: mol_type = other RNA
tgaagtaccagctactcgagaggctgaggcaggagaatcgcttgaacccaggaggtggagggtacagtaagccaagattgtgccactgcactccagcctggtgacagagcgagactctgtctaaaaaaaataaataaataatagaggtgaatgtctgcattaggatcaagacaagaagaagacagacaatcactttggaattctgagactacctccaagaatcatccacggaaggatgtcagccatttaaccagggctacggatcaaaaaggaaaaaatacagtcagtggacaagtagaagagtctcctgaaaaatatccgtatttgaaaaggcagcaggagttgatagaaaacataactaaaaaagtagaagacactgttaaatttgaatctggatcctatatagcttcttctctgggatctactgaggagtgaaatctaaatgaagatttagcttagaaagcatgaagatagtatgttccaattttaaataaaaattatattgtctgaaagacaatacaattttagtactgggggaaaaaaaactagattgttatttgaagaagaaaacatcatggttctctccaggtttaaaatgggtgctcccatgtaggctgattttcccggcatttgatcttaacttgaaggccatctgcccagcccagcaatcaaagggctgctaagctgtccttggtagcctctactgggcaaagctgtgctataactctgaagaaagggagatcttttaatgttgattactgaaaggcttagaaagatgtcttgaaagaggactaaacacaagaaaaataaatttttagcatttgagacttaggtgtttaagagtgcttagctcttaactattaactcttctgaggggagaaagctccatgaaacaggtttctgtttgaggctgtaattcttctagggcaagaacatctactcaacactaacaaatgctggaagcaggcatctgatttcctttgtgctaagggctgaaatcaatactggcctctggctccctacattcctatagaaccagctgcaggtaggcaggaagagaacaaaagttgttttggcggcactcagtacaataaaccgaagacaaaaaagacagagtaaagtctattaacagatggtaagtagtagatgatactggggttatttcggtaaaagaatatcagatttttatgaatgtcttaaatattacctataaccacagcagccacatgccccaggtttctcagaaccaatctcagtaccaaatattgtcatgttctttgtccacatactaggtttttggttttaaaaataaggtcgctgcagtttacatgcccactgctactgggaggcatacactgggccacttggataggctgtcattttctgcaaatcaagagacccatatcacctcctcaggagctctggcctatttttgtcctattcttgtctaccctaattgatatccttggctacatttatgataaatgtttcctgaccatcctttccttcttttagataccgatcagattaagtacaagcaattgtcaattatccagcacttgatctaggcctttaattccttcagagagagaaggaatatagagataaaactcccacccacttgaggtatggtttatgagctcttgcccaatcacattaccattcagaaggattttcctggctgacttaaaccaaaagcttcattgttccagtctgtcatgtcactgcagcaacagctgtcacctcaattatgcagtataatttttgacataatttatataagcacacagaattcaatcagcagctgagcagggaagcaatgttaacaaatgctatgaatgggtatatgatttgcatattatgtggctcatctgtggactggagcaatccatccattcccctcattactctgaataatctagaaatggtagatgctcctggccagacagctgtatgttttaaaaatcaaaaacaacaagaaaagcagcctcatggctggtgcgctctagaattaaggctatattaagcatttattcttatttcctcagctttggggctgggacaaggatcctcaaaaccctgctatttccttacttttaattgtgattctctagccctcctcaactacaaaaagaaaaggataaagtagggcatttcttgggggacaaaggcagaaggatatgatcagacaaatttctcaatagcaacacaagaagaaaccaaaacgaagtattttgctgagtaagaagaaaagggtgtgtcaacatgctaatgccagggcctgtcactttccaaggtgacagtctttcaggaacatgcctttatttttatttatattttttagagacagggggtctcactacattgcccaggctggtctcaaacttctggcttcaagcaattctcctgcctcagcctcccaaagtgctgggattacaggcggtagccactgtgcctggccatgaaaattcattttaaaaaataagatacaactataagtttgagggtagaaaaagggaagagcattaatattttggggactcttggtggtaaatccaggagccaagaatgcaggagacataactgctatgaacacttaaaattgatattgtggccaacagctcacctctaaaacttccccactgaaaataatggcatggaagggaaactcgggtccactgagaagtgagggtcaggtttgaagcctctttggtaacaggaatgctttgggaggccacaaaagttggcagggttggagggtgcctagcaccttggcacaagcaagcaccaggcaatcactcacacctacataaatatacagtctaaatatgaggaatggaaagaaatcatacatacataccatatatgataataaagacaattgtaccctaccccatcatcctcatgtactatagctacaaatctgcacagttaataatcttgtcattttatcacaaattgatatcactttacagaagcagaagtggggagtgctaaaagcaataccgaaagtcctggggctaaaaagagtgtcttgacagatttcagtgtaaaatttcaaatcttccaaaggatggagtaattctgggaggatgagtgaggatgaacaacagagggtggcccagaagaccacaccagaaaccctgtattctcctgggtagagctgaacaaggttgggaaagccccaacaggtaggcagttgctattggctttttaacagatgggcaacatcctttccatctcaacatgtcagaacaaaggccagctagtcagcaacatgttctaagaaccaaagcaagaaaccaaaattcaacatcattgtaacaaaatcccccaacctaaaaagcgaccaaccctgaaaagatcaagactctaaggtgattaaaaagttgaaactcatcttgaggtcacagggaagcagaaggaagagatcagggcaaaggaaaaaaaaattgtgggtattacactcagtatgtaaatgcctggtcttcacagagagacacttatcattaatcagaccatcagttatgttacaagagaaccaataccaacatttctcctgtggagcacagtgataagcacattttttatggatgtgtttaggatagaaaggggtgggtagaaaggagaggaggcagggaggtgaatgtattatgtacaaagagaaatgacagagaccatcccctcctttagctctttgctgtttctttctctttgttttccgcatcctcaggatatgcatgccatgtcagtctctcttcataaaatgctatcacaatttgtggacatttcacattagcttcttttgcaagaaccaggtcagcttcatctgtgtctttccatttcattaggaacattaaatcaccacaggaatctgttgccccaatgatcttttctggttccagtcctctctcaaagccccgagcgatatcattgctctgctctctcttttttttagatttgatgtcatcggcactgtttgagaaattggatttcctcttgttactttctgacttctccctgggtttattattttcaccctccttcatcttcttatactttttcataaattcagaaattagctcagggcaatccaagtttttctcaggttcccaagtattgtgctcctcagaaaagcctttccacttcagtagatattccacttgtcccttaaccacgcgcctgtctagcaccttctccacaacatactcctcctcatcctctgaagaagaactgtcagctgtccgcttggttttctttcccatgtcgcacaccgttccacctgaaagactaaggccaccaggtccccgggattgagagtgatcactcacgctaacgtctgccctgttcctgtatggtgaggccgcaccacaagccaccaccgccgccgccttctgcgcaacgccaaccgcccgccaaaac

SEQ ID NO: 18275 - RNA, 4385 nt, Homo sapiens
  source 1..4385: mol_type = other RNA
tgaagtaccagctactcgagaggctgaggcaggagaatcgcttgaacccaggaggtggagggtacagtaagccaagattgtgccactgcactccagcctggtgacagagcgagactctgtctaaaaaaaataaataaataatagaggtgaatgtctgcattaggatcaagacaagaagaagacagacaatcactttggaattctgagactacctccaagaatcatccacggaaggatgtcagccatttaaccagggctacggatcaaaaaggaaaaaatacagtcagtggacaagtagaagagtctcctgaaaaatatccgtatttgaaaaggcagcaggagttgatagaaaacataactaaaaaagtagaagacactgttaaatttgaatctggatcctatatagcttcttctctgggatctactgaggagtgaaatctaaatgaagatttagcttagaaagcatgaagatagtatgttccaattttaaataaaaattatattgtctgaaagacaatacaattttagtactgggggaaaaaaaactagattgttatttgaagaagaaaacatcatggttctctccaggtttaaaatgggtgctcccatgtaggctgattttcccggcatttgatcttaacttgaaggccatctgcccagcccagcaatcaaagggctgctaagctgtccttggtagcctctactgggcaaagctgtgctataactctgaagaaagggagatcttttaatgttgattactgaaaggcttagaaagatgtcttgaaagaggactaaacacaagaaaaataaatttttagcatttgagacttaggtgtttaagagtgcttagctcttaactattaactcttctgaggggagaaagctccatgaaacaggtttctgtttgaggctgtaattcttctagggcaagaacatctactcaacactaacaaatgctggaagcaggcatctgatttcctttgtgctaagggctgaaatcaatactggcctctggctccctacattcctatagaaccagctgcaggtaggcaggaagagaacaaaagttgttttggcggcactcagtacaataaaccgaagacaaaaaagacagagtaaagtctattaacagatggtaagtagtagatgatactggggttatttcggtaaaagaatatcagatttttatgaatgtcttaaatattacctataaccacagcagccacatgccccaggtttctcagaaccaatctcagtaccaaatattgtcatgttctttgtccacatactaggtttttggttttaaaaataaggtcgctgcagtttacatgcccactgctactgggaggcatacactgggccacttggataggctgtcattttctgcaaatcaagagacccatatcacctcctcaggagctctggcctatttttgtcctattcttgtctaccctaattgatatccttggctacatttatgataaatgtttcctgaccatcctttccttcttttagataccgatcagattaagtacaagcaattgtcaattatccagcacttgatctaggcctttaattccttcagagagagaaggaatatagagataaaactcccacccacttgaggtatggtttatgagctcttgcccaatcacattaccattcagaaggattttcctggctgacttaaaccaaaagcttcattgttccagtctgtcatgtcactgcagcaacagctgtcacctcaattatgcagtataatttttgacataatttatataagcacacagaattcaatcagcagctgagcagggaagcaatgttaacaaatgctatgaatgggtatatgatttgcatattatgtggctcatctgtggactggagcaatccatccattcccctcattactctgaataatctagaaatggtagatgctcctggccagacagctgtatgttttaaaaatcaaaaacaacaagaaaagcagcctcatggctggtgcgctctagaattaaggctatattaagcatttattcttatttcctcagctttggggctgggacaaggatcctcaaaaccctgctatttccttacttttaattgtgattctctagccctcctcaactacaaaaagaaaaggataaagtagggcatttcttgggggacaaaggcagaaggatatgatcagacaaatttctcaatagcaacacaagaagaaaccaaaacgaagtattttgctgagtaagaagaaaagggtgtgtcaacatgctaatgccagggcctgtcactttccaaggtgacagtctttcaggaacatgcctttatttttatttatattttttagagacagggggtctcactacattgcccaggctggtctcaaacttctggcttcaagcaattctcctgcctcagcctcccaaagtgctgggattacaggcggtagccactgtgcctggccatgaaaattcattttaaaaaataagatacaactataagtttgagggtagaaaaagggaagagcattaatattttggggactcttggtggtaaatccaggagccaagaatgcaggagacataactgctatgaacacttaaaattgatattgtggccaacagctcacctctaaaacttccccactgaaaataatggcatggaagggaaactcgggtccactgagaagtgagggtcaggtttgaagcctctttggtaacaggaatgctttgggaggccacaaaagttggcagggttggagggtgcctagcaccttggcacaagcaagcaccaggcaatcactcacacctacataaatatacagtctaaatatgaggaatggaaagaaatcatacatacataccatatatgataataaagacaattgtaccctaccccatcatcctcatgtactatagctacaaatctgcacagttaataatcttgtcattttatcacaaattgatatcactttacagaagcagaagtggggagtgctaaaagcaataccgaaagtcctggggctaaaaagagtgtcttgacagatttcagtgtaaaatttcaaatcttccaaaggatggagtaattctgggaggatgagtgaggatgaacaacagagggtggcccagaagaccacaccagaaaccctgtattctcctgggtagagctgaacaaggttgggaaagccccaacaggtaggcagttgctattggctttttaacagatgggcaacatcctttccatctcaacatgtcagaacaaaggccagctagtcagcaacatgttctaagaaccaaagcaagaaaccaaaattcaacatcattgtaacaaaatcccccaacctaaaaagcgaccaaccctgaaaagatcaagactctaaggtgattaaaaagttgaaactcatcttgaggtcacagggaagcagaaggaagagatcagggcaaaggaaaaaaaaattgtgggtattacactcagtatgtaaatgcctggtcttcacagagagacacttatcattaatcagaccatcagttatgttacaagagaaccaataccaacatttctcctgtggagcacagtgataagcacattttttatggatgtgtttaggatagaaaggggtgggtagaaaggagaggaggcagggaggtgaatgtattatgtacaaagagaaatgacagagaccatcccctcctttagctctttgctgtttctttctctttgttttccgcatcctcaggatatgcatgccatgtcagtctctcttcataaaatgctatcacaatttgtggacatttcacattagcttcttttgcaagaaccaggtcagcttcatctgtgtctttccatttcattaggaacattaaatcaccacaggaatctgttgccccaatgatcttttctggttccagtcctctctcaaagccccgagcgatatcattgctctgctctctcttttttttagatttgatgtcatcggcactgtttgagaaattggatttcctcttgttactttctgacttctccctgggtttattattttcaccctccttcatcttcttatactttttcataaattcagaaattagctcagggcaatccaagtttttctcaggttcccaagtattgtgctcctcagaaaagcctttccacttcagtagatattccacttgtcccttaaccacgcgcctgtctagcaccttctccacaacatactcctcctcatcctctgaagaagaactgtcagctgtccgcttggttttctttcccatgtcgcacaccgttccacctgaaagactaaggccaccaggtcccggatcgccccagttctttctttccctctgggctaacaggaggggcctcccctcccaggtctgggtcttggcgggctg

SEQ ID NO: 18276 - RNA, 4583 nt, Homo sapiens
  source 1..4583: mol_type = other RNA
tgaagtaccagctactcgagaggctgaggcaggagaatcgcttgaacccaggaggtggagggtacagtaagccaagattgtgccactgcactccagcctggtgacagagcgagactctgtctaaaaaaaataaataaataatagaggtgaatgtctgcattaggatcaagacaagaagaagacagacaatcactttggaattctgagactacctccaagaatcatccacggaaggatgtcagccatttaaccagggctacggatcaaaaaggaaaaaatacagtcagtggacaagtagaagagtctcctgaaaaatatccgtatttgaaaaggcagcaggagttgatagaaaacataactaaaaaagtagaagacactgttaaatttgaatctggatcctatatagcttcttctctgggatctactgaggagtgaaatctaaatgaagatttagcttagaaagcatgaagatagtatgttccaattttaaataaaaattatattgtctgaaagacaatacaattttagtactgggggaaaaaaaactagattgttatttgaagaagaaaacatcatggttctctccaggtttaaaatgggtgctcccatgtaggctgattttcccggcatttgatcttaacttgaaggccatctgcccagcccagcaatcaaagggctgctaagctgtccttggtagcctctactgggcaaagctgtgctataactctgaagaaagggagatcttttaatgttgattactgaaaggcttagaaagatgtcttgaaagaggactaaacacaagaaaaataaatttttagcatttgagacttaggtgtttaagagtgcttagctcttaactattaactcttctgaggggagaaagctccatgaaacaggtttctgtttgaggctgtaattcttctagggcaagaacatctactcaacactaacaaatgctggaagcaggcatctgatttcctttgtgctaagggctgaaatcaatactggcctctggctccctacattcctatagaaccagctgcaggtaggcaggaagagaacaaaagttgttttggcggcactcagtacaataaaccgaagacaaaaaagacagagtaaagtctattaacagatggtaagtagtagatgatactggggttatttcggtaaaagaatatcagatttttatgaatgtcttaaatattacctataaccacagcagccacatgccccaggtttctcagaaccaatctcagtaccaaatattgtcatgttctttgtccacatactaggtttttggttttaaaaataaggtcgctgcagtttacatgcccactgctactgggaggcatacactgggccacttggataggctgtcattttctgcaaatcaagagacccatatcacctcctcaggagctctggcctatttttgtcctattcttgtctaccctaattgatatccttggctacatttatgataaatgtttcctgaccatcctttccttcttttagataccgatcagattaagtacaagcaattgtcaattatccagcacttgatctaggcctttaattccttcagagagagaaggaatatagagataaaactcccacccacttgaggtatggtttatgagctcttgcccaatcacattaccattcagaaggattttcctggctgacttaaaccaaaagcttcattgttccagtctgtcatgtcactgcagcaacagctgtcacctcaattatgcagtataatttttgacataatttatataagcacacagaattcaatcagcagctgagcagggaagcaatgttaacaaatgctatgaatgggtatatgatttgcatattatgtggctcatctgtggactggagcaatccatccattcccctcattactctgaataatctagaaatggtagatgctcctggccagacagctgtatgttttaaaaatcaaaaacaacaagaaaagcagcctcatggctggtgcgctctagaattaaggctatattaagcatttattcttatttcctcagctttggggctgggacaaggatcctcaaaaccctgctatttccttacttttaattgtgattctctagccctcctcaactacaaaaagaaaaggataaagtagggcatttcttgggggacaaaggcagaaggatatgatcagacaaatttctcaatagcaacacaagaagaaaccaaaacgaagtattttgctgagtaagaagaaaagggtgtgtcaacatgctaatgccagggcctgtcactttccaaggtgacagtctttcaggaacatgcctttatttttatttatattttttagagacagggggtctcactacattgcccaggctggtctcaaacttctggcttcaagcaattctcctgcctcagcctcccaaagtgctgggattacaggcggtagccactgtgcctggccatgaaaattcattttaaaaaataagatacaactataagtttgagggtagaaaaagggaagagcattaatattttggggactcttggtggtaaatccaggagccaagaatgcaggagacataactgctatgaacacttaaaattgatattgtggccaacagctcacctctaaaacttccccactgaaaataatggcatggaagggaaactcgggtccactgagaagtgagggtcaggtttgaagcctctttggtaacaggaatgctttgggaggccacaaaagttggcagggttggagggtgcctagcaccttggcacaagcaagcaccaggcaatcactcacacctacataaatatacagtctaaatatgaggaatggaaagaaatcatacatacataccatatatgataataaagacaattgtaccctaccccatcatcctcatgtactatagctacaaatctgcacagttaataatcttgtcattttatcacaaattgatatcactttacagaagcagaagtggggagtgctaaaagcaataccgaaagtcctggggctaaaaagagtgtcttgacagatttcagtgtaaaatttcaaatcttccaaaggatggagtaattctgggaggatgagtgaggatgaacaacagagggtggcccagaagaccacaccagaaaccctgtattctcctgggtagagctgaacaaggttgggaaagccccaacaggtaggcagttgctattggctttttaacagatgggcaacatcctttccatctcaacatgtcagaacaaaggccagctagtcagcaacatgttctaagaaccaaagcaagaaaccaaaattcaacatcattgtaacaaaatcccccaacctaaaaagcgaccaaccctgaaaagatcaagactctaaggtgattaaaaagttgaaactcatcttgaggtcacagggaagcagaaggaagagatcagggcaaaggaaaaaaaaattgtgggtattacactcagtatgtaaatgcctggtcttcacagagagacacttatcattaatcagaccatcagttatgttacaagagaaccaataccaacatttctcctgtggagcacagtgataagcacattttttatggatgtgtttaggatagaaaggggtgggtagaaaggagaggaggcagggaggtgaatgtattatgtacaaagagaaatgacagagaccatcccctcctttagctctttgctgtttctttctctttgttttccgcatcctcaggatatgcatgccatgtcagtctctcttcataaaatgctatcacaatttgtggacatttcacattagcttcttttgcaagaaccaggtcagcttcatctgtgtctttccatttcattaggaacattaaatcaccacaggaatctgttgccccaatgatcttttctggttccagtcctctctcaaagccccgagcgatatcattgctctgctctctcttttttttagatttgatgtcatcggcactgtttgagaaattggatttcctcttgttactttctgacttctccctgggtttattattttcaccctccttcatcttcttatactttttcataaattcagaaattagctcagggcaatccaagtttttctcaggttcccaagtattgtgctcctcagaaaagcctttccacttcagtagatattccacttgtcccttaaccacgcgcctgtctagcaccttctccacaacatactcctcctcatcctctgaagaagaactgtcagctgtccgcttggttttctttcccatgtcgcacaccgttccacctgaaagactaaggccaccaggtcccttggaatttccgggagctgagcagtttaggtcagagcgctggggttaaaaccagccccatgttagatgcatgcagttaagcattgtggctatggcctcccctgcctcaccaggaaaaacaaggatttacatgtgttcttcattttgagggagagacaaggaaaatctccctttataccttcatgcagaagaggagccccaaaggtagaaaatgaatgggggttccctcctttacctaccggatcgccccagttctttctttccctctgggctaac

SEQ ID NO: 18277 - RNA, 6063 nt, Homo sapiens
  source 1..6063: mol_type = other RNA
tgaagtaccagctactcgagaggctgaggcaggagaatcgcttgaacccgggaggtggaggttgcggtgagccgagatcgtgccactgcactccagcctggcaacagagcaagactccttctaggggggaaaaaaaagggcatttcttcctattcaatgagaacatgaggaaaaggcaaaaggcagaggctggctgggagtgggtttgtgtgtgtaaaattgagtttcagtataaaaaaagatcaaggcaggactgaaagccctgaggctggcatcgcagctccagagcgaggggcaagcgtagggcgaggagcgaggatagggcgagggcgggagtagagcgaggggtaaggctagggtgagcacaggtggcaggggactctggtgggcctggactctggtgggcggggtgacccaggagctcggatgaagctcctacgggctccaggaaggttccctcaagtgccttccccacccaacccctaggccctgaacagagtcgagacccaggaatgtcccacgccccatcgcttcacctgtcccagggagaaattctggggttttttccacttcagccctctctgggggaagacgtcgggtcagaagcacatctgctcctgagagccagccgggagcaccaccatgactcttgcttagccaaacctgagggatctgaacctcctcctaggcccatccgtgcatgcccttgtaaaatcctttcagcaaatgaaccccgccgccatcccccccaacccccgccaccctcacatctgataggcttcttcagcctccaccatccccaggtgacctctgatcaccctggcctgccttcagcaagaatcctgctaggtgggtttagccgaaaacccccggacccctgaggtttgctcttagtgattttccatccactgatggtacctgtacctgtctcgatggtcctgaataaagtcttcctcacggccatttaacaagctcgccatcccactgtggggagagagacacatctgctgtagaaagagtgatacacacacagtggggggagccctcaatcggggacaacagcaggctcccagcattctcccagcgttcaaccgtgtatgtcactaagctcaggtgcttgggcctcatgggggactcctacacagcagctcctgctgagcactttggtggctggaatattctagaaagaggaataaagtaggagacacgagatctgtggtgctactttgtaattcgcactgtagggaaaagaagatgccgaagatgctgtagttaagccccaaatttatgtgcaagcctctgggtttttgtcttgtttttcaatcctgtcttctctgttttgccaaatgaggaaatggtggggagaattaaagcctcacacctttaacccctccactggactaatccaactgtatcattttatcttcgtcctcagcttttttgaagagaaagggagtgcaggctccgcagtgcgaaatcgtgaaacttatccttaatttggtgaatggagggtctgacaagtgaggggcccaggagctatgaccctgtggggagaccaagattggcaagagggaggctcggctcgcctcccctttccatgtgatcccacccagagctgccgccttcagctggctctctgtgccctgtggggctcccccatcacaaccgcctagagcagcagggtctcggacagcccaagcgtaagggacgcttgctgctgcctggggacagcaccccctcccccggtaacagtccccatttcctcctgggaaatgactctcccacaacatacccaggccgggtgtgagaagagggcttcccctccctggctaagcaagggggatgctcctctgcaactgaatctggaaccggctgaccccaaagttcctgtgtccctgggacccacctcttcctgcatggtgtggtcagcaattcctccatcaagcccccgacaaccctccagacaccctggtctgcaggggcaagtggaggccagagaacgctccgacacaggtcatgacccaattcacagcaagaaacagaaccccaacctcacatcaccccaacagcactccttttgctctgcaatccccaggtgacgtaggtctgtccaccagggagtgggcacacagggtggccacgacgctgctcggacaccgcagtcatgtccctctcagtggcctccaacactccactggctgggtgctccctggaccccgacccataacaagtgtccctgtgatgtagctgtctggccccaccctgagcccagagcgtcccccgggcagaaggggcaagaagtctgaccccaggggcctggccccacacagccttcaccccagcacctctgagacaagagctgtcggagtcactgagggagcgaacccagccgtcaggacttgaccccaggggatcacggagggagactccacatggaagaacagcctgttcggcttaaaacagacatggccagatccccatccctgaggccctggctgtggggcctgcaacaagctgtcacctagccctggagatgacagcaacacccccctcacaaggcggcccgaggattctcccggatagtctcaccaggtgtggtccagcccaggacaagagcacacagaggaaaacagcacacagaggacaaccaggaggcgcctggtggtccactcagctcagccggcagaggctgacccggctttccaggagtgcagggatggattagtgatgcttgcggtgggcccgggcgatggcgacggtgacctgtgttgcacatgtgccatctctcaggattcttctcctccctgaaccccagtgcactctctgacctcatcctggtgtcccctcaacacaagagcaaggcctcctgcaccggaagcgtctggccatgagtggcctcccgaccacctggacctgtgtgggctacagctccgccaggcctcgcacagtccaccctcaacccagccatcccttgacctgggagggtcagggaaatcagggcttctgagacagaggggctggttgccagccacccccgagaaagagatgtgacctgagccctgggtccctggatgaaggggctctgggggacacacgaaatcacagatgggaatctgggagtgccaagcccgtgggaattgccatttattcccaaagttgccaaaatcatcaccaaggattcaccgagggtgcgtgagcgggtgcgtgaggggaacgaggaggctcaaacactgactgggggttgggagtttggagggagggggaatgggtgggggccccagccacccctcccccttctaatgccacgggaaaggggtcctcctctggccagctcccctccccaggccccatgtccagtttctctccggggaggtggggtgggaaaggaagagggtgtagtgtgagtgggccccaggaaggggaagggcactgggggtggggatcccccatttcacatgcactcacaacactgatctcccagggagccggaatggggcagccggatggagccaggcccccttccgccctggattataggaggaagggattagtgttgggggccggggggcccgggggcatcatggggggcaggccagggcccccgccaaggggagagatgtacgtgggtggcgctccagggacgggaggcacaggactgagacggagctggttcagggtgagcgtcgcgggaggcgcgggctggaaggggttggtgacggaagggccagtggctgggcctccgcctggcaggaaggggttggaggccttggctccaggcggcgtggggcccggccggctcaccagcgagtccaggtcgacgagggctgcattgggccccaggaatgactccggcgtcttccgggtggggggcgtgggagttggtgtggctgcaggtggggggctgcccacagcctcagccagagatcccctgaccccactcatgtcaaacgccccagggcttcgggccggcacctctcctgccagcagctccagctctcctgcgctgctcccggaggtcggcagtgccgtgcggagtcggtcaaagtcagagaactcgtcgggctccgtgtcgaatcccccggctgctgttgtgccattggtgctgggcttggcaggtgaccctccccagggatctgagaaggccggggccggtgtccagggatcggaggctgagggcccactgaccgggaccccaccatcggaacttccccatggatcaggcgtgggcccctccccagctgcaggggctggggtcccaccccaagggtcaactgagggtcctgcaggggcagcaggcctccaggggtccccagaggccggcgtgggggctggacctccccagggatcagcagctggagggacaggggggccgccccaggggtccgaggtgggggcagccgtggggacggcagcagccatgggtgctgggcccccccaggggtctgtggtcggggcaggagctggggccgtgaagacgtcagcaaggtccatgagggacgactcctccttgcccccagtctccctcttgctctcctcgattgccatctgcagccgcaggtcatccccgcgacggatccgctcctcctggtcggcctcctccttgctcatggccagggccagctggagctgcagctcctcctccccgctgctctgcggccacgcctgctccgcctcgggaggggggcctgagcccacagctgctgatgaggccgtggcggtctgtgccagcttttccttggtcttgagcgcgtgcgcccgctcttcccgcagccggtcctcgtcgcgcagcagggccaccagctgcttagctttctcacgcacgttcacgccctggtccttgccgtcgcggtccacgtactggaagtccttcagcgtctgcacggcgtacatgttctccttgcactgctgcgacacgcgctccgagccggtcttgatgaggtactccatcagcgtcatggccttgtaaacgtgacgccagttcttgccatggtcattgagccgcttccagatcatgctcatgatctccgagaaggcgacaacgttgtaggtgaggtcggcaatctctgacatgagggagctggatgggccccaggggtcattgctcgtggcctctcgaaccttgatctccgcctctgagtagttgtggacgatgttcttcatctggcgcctcaaggacgaggtcgacatggtgcccggctgcagcagcaaggggcacagggccccgatgcgtggagagatggggcgactcccggacgaaggctgcggcaggtgctggcaggtcaccgcatccagggcggcaggaagaaccggggaagccagaagaccagacgtcccaaggatagcggaagcccaaggctcaggagagataaggaacctaacagccccactgcctgggtccctgctgtgtgccaggtgctcgctcagcacaagagggacattacctttttcaacactgcatgcaaagactgggctccttactcctggagcagcctggttccagagccagctctgatcacccatctatgcggctccaagaagccacagagggagattttcaaagccccgccatgatgtaagcccaggggagatagggatgacggagagaggctggcctctgcttccacctcaggccagaaagccaggcacctgaagacagatgtagctagttaaaaagtaactctctggagtcccaaaacagccccagcctaatacattaagatgaagagatgatgtaacaaatgcagagaaggggactgagaagaaatagaagacagttctgacagaaagagacacatagaaacctgggcagagggagctaggcagagacacaatgagaaaaacacaggcagcagcagatacaagaacatgggaagacagggaggcaggaggccaaggaagaaagaggcccagaaacaaaaagagacctggcgctgagaaataagagataagaaaaatggaatctaatggcaaagaatataaaatgtgggttcaaatcctggccacatcagctacctgcagcgcacacctccttgagacacagtttgctcaactctgaaatgaaag

SEQ ID NO: 18278 - RNA, 5573 nt, Homo sapiens
  source 1..5573: mol_type = other RNA
tgaagtaccagctactcgagaggctgaggcaggagaatcgcttgaacccgggaggtggaggttgcggtgagccgagatcgtgccactgcactccagcctggcaacagagcaagactccttctaggggggaaaaaaaagggcatttcttcctattcaatgagaacatgaggaaaaggcaaaaggcagaggctggctgggagtgggtttgtgtgtgtaaaattgagtttcagtataaaaaaagatcaaggcaggactgaaagccctgaggctggcatcgcagctccagagcgaggggcaagcgtagggcgaggagcgaggatagggcgagggcgggagtagagcgaggggtaaggctagggtgagcacaggtggcaggggactctggtgggcctggactctggtgggcggggtgacccaggagctcggatgaagctcctacgggctccaggaaggttccctcaagtgccttccccacccaacccctaggccctgaacagagtcgagacccaggaatgtcccacgccccatcgcttcacctgtcccagggagaaattctggggttttttccacttcagccctctctgggggaagacgtcgggtcagaagcacatctgctcctgagagccagccgggagcaccaccatgactcttgcttagccaaacctgagggatctgaacctcctcctaggcccatccgtgcatgcccttgtaaaatcctttcagcaaatgaaccccgccgccatcccccccaacccccgccaccctcacatctgataggcttcttcagcctccaccatccccaggtgacctctgatcaccctggcctgccttcagcaagaatcctgctaggtgggtttagccgaaaacccccggacccctgaggtttgctcttagtgattttccatccactgatggtacctgtacctgtctcgatggtcctgaataaagtcttcctcacggccatttaacaagctcgccatcccactgtggggagagagacacatctgctgtagaaagagtgatacacacacagtggggggagccctcaatcggggacaacagcaggctcccagcattctcccagcgttcaaccgtgtatgtcactaagctcaggtgcttgggcctcatgggggactcctacacagcagctcctgctgagcactttggtggctggaatattctagaaagaggaataaagtaggagacacgagatctgtggtgctactttgtaattcgcactgtagggaaaagaagatgccgaagatgctgtagttaagccccaaatttatgtgcaagcctctgggtttttgtcttgtttttcaatcctgtcttctctgttttgccaaatgaggaaatggtggggagaattaaagcctcacacctttaacccctccactggactaatccaactgtatcattttatcttcgtcctcagcttttttgaagagaaagggagtgcaggctccgcagtgcgaaatcgtgaaacttatccttaatttggtgaatggagggtctgacaagtgaggggcccaggagctatgaccctgtggggagaccaagattggcaagagggaggctcggctcgcctcccctttccatgtgatcccacccagagctgccgccttcagctggctctctgtgccctgtggggctcccccatcacaaccgcctagagcagcagggtctcggacagcccaagcgtaagggacgcttgctgctgcctggggacagcaccccctcccccggtaacagtccccatttcctcctgggaaatgactctcccacaacatacccaggccgggtgtgagaagagggcttcccctccctggctaagcaagggggatgctcctctgcaactgaatctggaaccggctgaccccaaagttcctgtgtccctgggacccacctcttcctgcatggtgtggtcagcaattcctccatcaagcccccgacaaccctccagacaccctggtctgcaggggcaagtggaggccagagaacgctccgacacaggtcatgacccaattcacagcaagaaacagaaccccaacctcacatcaccccaacagcactccttttgctctgcaatccccaggtgacgtaggtctgtccaccagggagtgggcacacagggtggccacgacgctgctcggacaccgcagtcatgtccctctcagtggcctccaacactccactggctgggtgctccctggaccccgacccataacaagtgtccctgtgatgtagctgtctggccccaccctgagcccagagcgtcccccgggcagaaggggcaagaagtctgaccccaggggcctggccccacacagccttcaccccagcacctctgagacaagagctgtcggagtcactgagggagcgaacccagccgtcaggacttgaccccaggggatcacggagggagactccacatggaagaacagcctgttcggcttaaaacagacatggccagatccccatccctgaggccctggctgtggggcctgcaacaagctgtcacctagccctggagatgacagcaacacccccctcacaaggcggcccgaggattctcccggatagtctcaccaggtgtggtccagcccaggacaagagcacacagaggaaaacagcacacagaggacaaccaggaggcgcctggtggtccactcagctcagccggcagaggctgacccggctttccaggagtgcagggatggattagtgatgcttgcggtgggcccgggcgatggcgacggtgacctgtgttgcacatgtgccatctctcaggattcttctcctccctgaaccccagtgcactctctgacctcatcctggtgtcccctcaacacaagagcaaggcctcctgcaccggaagcgtctggccatgagtggcctcccgaccacctggacctgtgtgggctacagctccgccaggcctcgcacagtccaccctcaacccagccatcccttgacctgggagggtcagggaaatcagggcttctgagacagaggggctggttgccagccacccccgagaaagagatgtgacctgagccctgggtccctggatgaaggggctctgggggacacacgaaatcacagatgggaatctgggagtgccaagcccgtgggaattgccatttattcccaaagttgccaaaatcatcaccaaggattcaccgagggtgcgtgagcgggtgcgtgaggggaacgaggaggctcaaacactgactgggggttgggagtttggagggagggggaatgggtgggggccccagccacccctcccccttctaatgccacgggaaaggggtcctcctctggccagctcccctccccaggccccatgtccagtttctctccggggaggtggggtgggaaaggaagagggtgtagtgtgagtgggccccaggaaggggaagggcactgggggtggggatcccccatttcacatgcactcacaacactgatctcccagggagccggaatggggcagccggatggagccaggcccccttccgccctggattataggaggaagggattagtgttgggggccggggggcccgggggcatcatggggggcaggccagggcccccgccaaggggagagatgtacgtgggtggcgctccagggacgggaggcacaggactgagacggagctggttcagggtgagcgtcgcgggaggcgcgggctggaaggggttggtgacggaagggccagtggctgggcctccgcctggcaggaaggggttggaggccttggctccaggcggcgtggggcccggccggctcaccagcgagtccaggtcgacgagggctgcattgggccccaggaatgactccggcgtcttccgggtggggggcgtgggagttggtgtggctgcaggtggggggctgcccacagcctcagccagagatcccctgaccccactcatgtcaaacgccccagggcttcgggccggcacctctcctgccagcagctccagctctcctgcgctgctcccggaggtcggcagtgccgtgcggagtcggtcaaagtcagagaactcgtcgggctccgtgtcgaatcccccggctgctgttgtgccattggtgctgggcttggcaggtgaccctccccagggatctgagaaggccggggccggtgtccagggatcggaggctgagggcccactgaccgggaccccaccatcggaacttccccatggatcaggcgtgggcccctccccagctgcaggggctggggtcccaccccaagggtcaactgagggtcctgcaggggcagcaggcctccaggggtccccagaggccggcgtgggggctggacctccccagggatcagcagctggagggacaggggggccgccccaggggtccgaggtgggggcagccgtggggacggcagcagccatgggtgctgggcccccccaggggtctgtggtcggggcaggagctggggccgtgaagacgtcagcaaggtccatgagggacgactcctccttgcccccagtctccctcttgctctcctcgattgccatctgcagccgcaggtcatccccgcgacggatccgctcctccttatcatgctcttctcggctcaaactaagggccagctggagctgggcgtcgtcctcggggccgcaggacgggggctggtcggcctcctccttgctcatggccagggccagctggagctgcagctcctcctccccgctgctctgcggccacgcctgctccgcctcgggaggggggcctgagcccacagctgctgatgaggccgtggcggtctgtgccagcttttccttggtcttgagcgcgtgcgcccgctcttcccgcagccggtcctcgtcgcgcagcagggccaccagctgcttagctttctcacgcacgttcacgccctggtccttgccgtcgcggtccacgtactggaagtccttcagcgtctgcacggcgtacatgttctccttgcactgctgcgacacgcgctccgagccggtcttgatgaggtactccatcagcgtcatggccttgtaaacgtgacgccagttcttgccatggtcattgagccgcttccagatcatgctcatgatctccgagaaggcgacaacgttgtaggtgaggtcggcaatctctgacatgagggagctggatgggccccaggggtcattgctcgtggcctctcgaaccttgatctccgcctctgagtagttgtggacgatgttcttcatctggcgcctcaaggacgaggtcgacatggtgcccggctgcagcagcaaggggcacagggccccgatgcgtggagagatggggcgactcccggacgaaggctgcggcaggtgctggcaggtcaccgcatctcggccccctcacgccgggctctggggggtcatggcggtcagccccctgccccgctcggcctcggtgtcgcgggacgtgcgccgggccacgggcgcacgcacgaacgcaaggagggccgcacgccgacggctccgccgccccgccgcccagaaggggcgcggagagccgggcgggggaggggagccgccgaggagacgggaagcaacag

SEQ ID NO: 18279 - RNA, 5495 nt, Homo sapiens
  source 1..5495: mol_type = other RNA
tgaagtaccagctactcgagaggctgaggcaggagaatcgcttgaacccgggaggtggaggttgcggtgagccgagatcgtgccactgcactccagcctggcaacagagcaagactccttctaggggggaaaaaaaagggcatttcttcctattcaatgagaacatgaggaaaaggcaaaaggcagaggctggctgggagtgggtttgtgtgtgtaaaattgagtttcagtataaaaaaagatcaaggcaggactgaaagccctgaggctggcatcgcagctccagagcgaggggcaagcgtagggcgaggagcgaggatagggcgagggcgggagtagagcgaggggtaaggctagggtgagcacaggtggcaggggactctggtgggcctggactctggtgggcggggtgacccaggagctcggatgaagctcctacgggctccaggaaggttccctcaagtgccttccccacccaacccctaggccctgaacagagtcgagacccaggaatgtcccacgccccatcgcttcacctgtcccagggagaaattctggggttttttccacttcagccctctctgggggaagacgtcgggtcagaagcacatctgctcctgagagccagccgggagcaccaccatgactcttgcttagccaaacctgagggatctgaacctcctcctaggcccatccgtgcatgcccttgtaaaatcctttcagcaaatgaaccccgccgccatcccccccaacccccgccaccctcacatctgataggcttcttcagcctccaccatccccaggtgacctctgatcaccctggcctgccttcagcaagaatcctgctaggtgggtttagccgaaaacccccggacccctgaggtttgctcttagtgattttccatccactgatggtacctgtacctgtctcgatggtcctgaataaagtcttcctcacggccatttaacaagctcgccatcccactgtggggagagagacacatctgctgtagaaagagtgatacacacacagtggggggagccctcaatcggggacaacagcaggctcccagcattctcccagcgttcaaccgtgtatgtcactaagctcaggtgcttgggcctcatgggggactcctacacagcagctcctgctgagcactttggtggctggaatattctagaaagaggaataaagtaggagacacgagatctgtggtgctactttgtaattcgcactgtagggaaaagaagatgccgaagatgctgtagttaagccccaaatttatgtgcaagcctctgggtttttgtcttgtttttcaatcctgtcttctctgttttgccaaatgaggaaatggtggggagaattaaagcctcacacctttaacccctccactggactaatccaactgtatcattttatcttcgtcctcagcttttttgaagagaaagggagtgcaggctccgcagtgcgaaatcgtgaaacttatccttaatttggtgaatggagggtctgacaagtgaggggcccaggagctatgaccctgtggggagaccaagattggcaagagggaggctcggctcgcctcccctttccatgtgatcccacccagagctgccgccttcagctggctctctgtgccctgtggggctcccccatcacaaccgcctagagcagcagggtctcggacagcccaagcgtaagggacgcttgctgctgcctggggacagcaccccctcccccggtaacagtccccatttcctcctgggaaatgactctcccacaacatacccaggccgggtgtgagaagagggcttcccctccctggctaagcaagggggatgctcctctgcaactgaatctggaaccggctgaccccaaagttcctgtgtccctgggacccacctcttcctgcatggtgtggtcagcaattcctccatcaagcccccgacaaccctccagacaccctggtctgcaggggcaagtggaggccagagaacgctccgacacaggtcatgacccaattcacagcaagaaacagaaccccaacctcacatcaccccaacagcactccttttgctctgcaatccccaggtgacgtaggtctgtccaccagggagtgggcacacagggtggccacgacgctgctcggacaccgcagtcatgtccctctcagtggcctccaacactccactggctgggtgctccctggaccccgacccataacaagtgtccctgtgatgtagctgtctggccccaccctgagcccagagcgtcccccgggcagaaggggcaagaagtctgaccccaggggcctggccccacacagccttcaccccagcacctctgagacaagagctgtcggagtcactgagggagcgaacccagccgtcaggacttgaccccaggggatcacggagggagactccacatggaagaacagcctgttcggcttaaaacagacatggccagatccccatccctgaggccctggctgtggggcctgcaacaagctgtcacctagccctggagatgacagcaacacccccctcacaaggcggcccgaggattctcccggatagtctcaccaggtgtggtccagcccaggacaagagcacacagaggaaaacagcacacagaggacaaccaggaggcgcctggtggtccactcagctcagccggcagaggctgacccggctttccaggagtgcagggatggattagtgatgcttgcggtgggcccgggcgatggcgacggtgacctgtgttgcacatgtgccatctctcaggattcttctcctccctgaaccccagtgcactctctgacctcatcctggtgtcccctcaacacaagagcaaggcctcctgcaccggaagcgtctggccatgagtggcctcccgaccacctggacctgtgtgggctacagctccgccaggcctcgcacagtccaccctcaacccagccatcccttgacctgggagggtcagggaaatcagggcttctgagacagaggggctggttgccagccacccccgagaaagagatgtgacctgagccctgggtccctggatgaaggggctctgggggacacacgaaatcacagatgggaatctgggagtgccaagcccgtgggaattgccatttattcccaaagttgccaaaatcatcaccaaggattcaccgagggtgcgtgagcgggtgcgtgaggggaacgaggaggctcaaacactgactgggggttgggagtttggagggagggggaatgggtgggggccccagccacccctcccccttctaatgccacgggaaaggggtcctcctctggccagctcccctccccaggccccatgtccagtttctctccggggaggtggggtgggaaaggaagagggtgtagtgtgagtgggccccaggaaggggaagggcactgggggtggggatcccccatttcacatgcactcacaacactgatctcccagggagccggaatggggcagccggatggagccaggcccccttccgccctggattataggaggaagggattagtgttgggggccggggggcccgggggcatcatggggggcaggccagggcccccgccaaggggagagatgtacgtgggtggcgctccagggacgggaggcacaggactgagacggagctggttcagggtgagcgtcgcgggaggcgcgggctggaaggggttggtgacggaagggccagtggctgggcctccgcctggcaggaaggggttggaggccttggctccaggcggcgtggggcccggccggctcaccagcgagtccaggtcgacgagggctgcattgggccccaggaatgactccggcgtcttccgggtggggggcgtgggagttggtgtggctgcaggtggggggctgcccacagcctcagccagagatcccctgaccccactcatgtcaaacgccccagggcttcgggccggcacctctcctgccagcagctccagctctcctgcgctgctcccggaggtcggcagtgccgtgcggagtcggtcaaagtcagagaactcgtcgggctccgtgtcgaatcccccggctgttgtgccattggtgctgggcttggcaggtgaccctccccagggatctgagaaggccggggccggtgtccagggatcggaggctgagggcccactgaccgggaccccaccatcggaacttccccatggatcaggcgtgggcccctccccagctgcaggggctggggtcccaccccaagggtcaactgagggtcctgcaggggcagcaggcctccaggggtccccagaggccggcgtgggggctggacctccccagggatcagcagctggagggacaggggggccgccccaggggtccgaggtgggggcagccgtggggacggcagcagccatgggtgctgggcccccccaggggtctgtggtcggggcaggagctggggccgtgaagacgtcagcaaggtccatgagggacgactcctccttgcccccagtctccctcttgctctcctcgattgccatctgcagccgcaggtcatccccgcgacggatccgctcctcctggtcggcctcctccttgctcatggccagggccagctggagctgcagctcctcctccccgctgctctgcggccacgcctgctccgcctcgggaggggggcctgagcccacagctgctgatgaggccgtggcggtctgtgccagcttttccttggtcttgagcgcgtgcgcccgctcttcccgcagccggtcctcgtcgcgcagcagggccaccagctgcttagctttctcacgcacgttcacgccctggtccttgccgtcgcggtccacgtactggaagtccttcagcgtctgcacggcgtacatgttctccttgcactgctgcgacacgcgctccgagccggtcttgatgaggtactccatcagcgtcatggccttgtaaacgtgacgccagttcttgccatggtcattgagccgcttccagatcatgctcatgatctccgagaaggcgacaacgttgtaggtgaggtcggcaatctctgacatgagggagctggatgggccccaggggtcattgctcgtggcctctcgaaccttgatctccgcctctgagtagttgtggacgatgttcttcatctggcgcctcaaggacgaggtcgacatggtgcccggctgcagcagcaaggggcacagggccccgatgcgtggagagatggggcgactcccggacgaaggctgcggcaggtgctggcaggtcaccgcatctcggccccctcacgccgggctctggggggtcatggcggtcagccccctgccccgctcggcctcggtgtcgcgggacgtgcgccgggccacgggcgcacgcacgaacgcaaggagggccgcacgccgacggctccgccgccccgccgcccagaaggggcgcggagagccgggcgggggaggggagccgccgaggagacgggaagcaacag

SEQ ID NO: 18280 - RNA, 5570 nt, Homo sapiens
  source 1..5570: mol_type = other RNA
tgaagtaccagctactcgagaggctgaggcaggagaatcgcttgaacccgggaggtggaggttgcggtgagccgagatcgtgccactgcactccagcctggcaacagagcaagactccttctaggggggaaaaaaaagggcatttcttcctattcaatgagaacatgaggaaaaggcaaaaggcagaggctggctgggagtgggtttgtgtgtgtaaaattgagtttcagtataaaaaaagatcaaggcaggactgaaagccctgaggctggcatcgcagctccagagcgaggggcaagcgtagggcgaggagcgaggatagggcgagggcgggagtagagcgaggggtaaggctagggtgagcacaggtggcaggggactctggtgggcctggactctggtgggcggggtgacccaggagctcggatgaagctcctacgggctccaggaaggttccctcaagtgccttccccacccaacccctaggccctgaacagagtcgagacccaggaatgtcccacgccccatcgcttcacctgtcccagggagaaattctggggttttttccacttcagccctctctgggggaagacgtcgggtcagaagcacatctgctcctgagagccagccgggagcaccaccatgactcttgcttagccaaacctgagggatctgaacctcctcctaggcccatccgtgcatgcccttgtaaaatcctttcagcaaatgaaccccgccgccatcccccccaacccccgccaccctcacatctgataggcttcttcagcctccaccatccccaggtgacctctgatcaccctggcctgccttcagcaagaatcctgctaggtgggtttagccgaaaacccccggacccctgaggtttgctcttagtgattttccatccactgatggtacctgtacctgtctcgatggtcctgaataaagtcttcctcacggccatttaacaagctcgccatcccactgtggggagagagacacatctgctgtagaaagagtgatacacacacagtggggggagccctcaatcggggacaacagcaggctcccagcattctcccagcgttcaaccgtgtatgtcactaagctcaggtgcttgggcctcatgggggactcctacacagcagctcctgctgagcactttggtggctggaatattctagaaagaggaataaagtaggagacacgagatctgtggtgctactttgtaattcgcactgtagggaaaagaagatgccgaagatgctgtagttaagccccaaatttatgtgcaagcctctgggtttttgtcttgtttttcaatcctgtcttctctgttttgccaaatgaggaaatggtggggagaattaaagcctcacacctttaacccctccactggactaatccaactgtatcattttatcttcgtcctcagcttttttgaagagaaagggagtgcaggctccgcagtgcgaaatcgtgaaacttatccttaatttggtgaatggagggtctgacaagtgaggggcccaggagctatgaccctgtggggagaccaagattggcaagagggaggctcggctcgcctcccctttccatgtgatcccacccagagctgccgccttcagctggctctctgtgccctgtggggctcccccatcacaaccgcctagagcagcagggtctcggacagcccaagcgtaagggacgcttgctgctgcctggggacagcaccccctcccccggtaacagtccccatttcctcctgggaaatgactctcccacaacatacccaggccgggtgtgagaagagggcttcccctccctggctaagcaagggggatgctcctctgcaactgaatctggaaccggctgaccccaaagttcctgtgtccctgggacccacctcttcctgcatggtgtggtcagcaattcctccatcaagcccccgacaaccctccagacaccctggtctgcaggggcaagtggaggccagagaacgctccgacacaggtcatgacccaattcacagcaagaaacagaaccccaacctcacatcaccccaacagcactccttttgctctgcaatccccaggtgacgtaggtctgtccaccagggagtgggcacacagggtggccacgacgctgctcggacaccgcagtcatgtccctctcagtggcctccaacactccactggctgggtgctccctggaccccgacccataacaagtgtccctgtgatgtagctgtctggccccaccctgagcccagagcgtcccccgggcagaaggggcaagaagtctgaccccaggggcctggccccacacagccttcaccccagcacctctgagacaagagctgtcggagtcactgagggagcgaacccagccgtcaggacttgaccccaggggatcacggagggagactccacatggaagaacagcctgttcggcttaaaacagacatggccagatccccatccctgaggccctggctgtggggcctgcaacaagctgtcacctagccctggagatgacagcaacacccccctcacaaggcggcccgaggattctcccggatagtctcaccaggtgtggtccagcccaggacaagagcacacagaggaaaacagcacacagaggacaaccaggaggcgcctggtggtccactcagctcagccggcagaggctgacccggctttccaggagtgcagggatggattagtgatgcttgcggtgggcccgggcgatggcgacggtgacctgtgttgcacatgtgccatctctcaggattcttctcctccctgaaccccagtgcactctctgacctcatcctggtgtcccctcaacacaagagcaaggcctcctgcaccggaagcgtctggccatgagtggcctcccgaccacctggacctgtgtgggctacagctccgccaggcctcgcacagtccaccctcaacccagccatcccttgacctgggagggtcagggaaatcagggcttctgagacagaggggctggttgccagccacccccgagaaagagatgtgacctgagccctgggtccctggatgaaggggctctgggggacacacgaaatcacagatgggaatctgggagtgccaagcccgtgggaattgccatttattcccaaagttgccaaaatcatcaccaaggattcaccgagggtgcgtgagcgggtgcgtgaggggaacgaggaggctcaaacactgactgggggttgggagtttggagggagggggaatgggtgggggccccagccacccctcccccttctaatgccacgggaaaggggtcctcctctggccagctcccctccccaggccccatgtccagtttctctccggggaggtggggtgggaaaggaagagggtgtagtgtgagtgggccccaggaaggggaagggcactgggggtggggatcccccatttcacatgcactcacaacactgatctcccagggagccggaatggggcagccggatggagccaggcccccttccgccctggattataggaggaagggattagtgttgggggccggggggcccgggggcatcatggggggcaggccagggcccccgccaaggggagagatgtacgtgggtggcgctccagggacgggaggcacaggactgagacggagctggttcagggtgagcgtcgcgggaggcgcgggctggaaggggttggtgacggaagggccagtggctgggcctccgcctggcaggaaggggttggaggccttggctccaggcggcgtggggcccggccggctcaccagcgagtccaggtcgacgagggctgcattgggccccaggaatgactccggcgtcttccgggtggggggcgtgggagttggtgtggctgcaggtggggggctgcccacagcctcagccagagatcccctgaccccactcatgtcaaacgccccagggcttcgggccggcacctctcctgccagcagctccagctctcctgcgctgctcccggaggtcggcagtgccgtgcggagtcggtcaaagtcagagaactcgtcgggctccgtgtcgaatcccccggctgttgtgccattggtgctgggcttggcaggtgaccctccccagggatctgagaaggccggggccggtgtccagggatcggaggctgagggcccactgaccgggaccccaccatcggaacttccccatggatcaggcgtgggcccctccccagctgcaggggctggggtcccaccccaagggtcaactgagggtcctgcaggggcagcaggcctccaggggtccccagaggccggcgtgggggctggacctccccagggatcagcagctggagggacaggggggccgccccaggggtccgaggtgggggcagccgtggggacggcagcagccatgggtgctgggcccccccaggggtctgtggtcggggcaggagctggggccgtgaagacgtcagcaaggtccatgagggacgactcctccttgcccccagtctccctcttgctctcctcgattgccatctgcagccgcaggtcatccccgcgacggatccgctcctccttatcatgctcttctcggctcaaactaagggccagctggagctgggcgtcgtcctcggggccgcaggacgggggctggtcggcctcctccttgctcatggccagggccagctggagctgcagctcctcctccccgctgctctgcggccacgcctgctccgcctcgggaggggggcctgagcccacagctgctgatgaggccgtggcggtctgtgccagcttttccttggtcttgagcgcgtgcgcccgctcttcccgcagccggtcctcgtcgcgcagcagggccaccagctgcttagctttctcacgcacgttcacgccctggtccttgccgtcgcggtccacgtactggaagtccttcagcgtctgcacggcgtacatgttctccttgcactgctgcgacacgcgctccgagccggtcttgatgaggtactccatcagcgtcatggccttgtaaacgtgacgccagttcttgccatggtcattgagccgcttccagatcatgctcatgatctccgagaaggcgacaacgttgtaggtgaggtcggcaatctctgacatgagggagctggatgggccccaggggtcattgctcgtggcctctcgaaccttgatctccgcctctgagtagttgtggacgatgttcttcatctggcgcctcaaggacgaggtcgacatggtgcccggctgcagcagcaaggggcacagggccccgatgcgtggagagatggggcgactcccggacgaaggctgcggcaggtgctggcaggtcaccgcatctcggccccctcacgccgggctctggggggtcatggcggtcagccccctgccccgctcggcctcggtgtcgcgggacgtgcgccgggccacgggcgcacgcacgaacgcaaggagggccgcacgccgacggctccgccgccccgccgcccagaaggggcgcggagagccgggcgggggaggggagccgccgaggagacgggaagcaacag

SEQ ID NO: 18281 - RNA, 370 nt, Homo sapiens
  source 1..370: mol_type = other RNA
tgaagtaccagctactcgagaggctgaggcaggagaatcgcttgaacctgggaggcagaggttgcagtgagccaagatcacaccactatactccagcctgggtgacagagcgagactccatcaatagcgagtggagaagagtattttgtcgaagtttgcaaaccaatctttgggagccagaggtgggaattttaaaatgaggtcttttccttggaattttcttaaagtggtatcgttgcctgttgatattgaagtttgtcaaagaacgtgaaatcaccagcttagaggatttttttccccccttcaagacgctaagcaaaagccactccgtcgacatcaaaccccacgccggagccggaagcaagagtag

SEQ ID NO: 18282 - RNA, 371 nt, Homo sapiens
  source 1..371: mol_type = other RNA
tgaagtaccagctactcgagaggctgaggcaggagaatcgcttgaacctgggaggcagaggttgcagtgagccaagatcacaccactatactccagcctgggtgacagagcgagactccatcaatagcgagtggagaagagtattttgtcgaagtttgcaaaccaatctttgggagccagaggtgggaattttaaaatgaggtcttttccttggaattttcttaaagtggtatcgttgcctgttgatattgaagtttgtcaaagaacgtgaaatcaccagcttagaggatttttttccccccttcaagacgctaagcaaaagccactccgtcgacatcaaaccccacgccggagccggaagcaagagtaga

SEQ ID NO: 18283 - RNA, 268 nt, Homo sapiens
  source 1..268: mol_type = other RNA
tgaagtaccagctactcgagaggctgaggcaggagaatcgcttgaacctgggaggcagaggttgcagtgagccaagatcacaccactatactccagcctgggtgacagagcgagactccatcgtttctttttcgagcgaattacacagttgtcttggcagcgtgatttgccctctggttcctgctttatcagtttggtgattctttgtacagattgataaccatgaaaaagtctaaagtagggcagttccggagcagccttttcccat

SEQ ID NO: 18284 - RNA, 286 nt, Homo sapiens
  source 1..286: mol_type = other RNA
tgaagtaccagctactcgagaggctgaggcaggagaatcgcttgaacctgggaggcagaggttgcagtgagccaagatcacaccactatactccagcctgggtgacagagcgagactccatcgtttctttttcgagcgaattacacagttgtcttggcagcgtgatttgccctctggttcctgctttatcagtttggtgattctttgtacagattgataaccatgaaaaagtctaaagtagggcagttccggagcagccttttcccataaagcaagcgggtacctc

SEQ ID NO: 18285 - RNA, 315 nt, Homo sapiens
  source 1..315: mol_type = other RNA
tgaagtaccagctactcgagaggctgaggcaggagaatcgcttgaacctgggaggcagaggttgcagtgagccaagatcacaccactatactccagcctgggtgacagagcgagactccatcgtttctttttcgagcgaattacacagttgtcttggcagcgtgatttgccctctggttcctgctttatcagtttggtgattctttgtacagattgataaccatgaaaaagtctaaagtagggcagttccggagcagccttttcccataaagcaagcgggtacctcacaaaactccaggcaaaagaatgaatgat

SEQ ID NO: 18286 - RNA, 318 nt, Homo sapiens
  source 1..318: mol_type = other RNA
tgaagtaccagctactcgagaggctgaggcaggagaatcgcttgaacctgggaggcagaggttgcagtgagccaagatcacaccactatactccagcctgggtgacagagcgagactccatcgtttctttttcgagcgaattacacagttgtcttggcagcgtgatttgccctctggttcctgctttatcagtttggtgattctttgtacagattgataaccatgaaaaagtctaaagtagggcagttccggagcagccttttcccataaagcaagcgggtacctcacaaaactccaggcaaaagaatgaatgataga

SEQ ID NO: 18287 - RNA, 576 nt, Homo sapiens
  source 1..576: mol_type = other RNA
tgaagtaccagctactcgagaggctgaggcaggagaatcgcttgaacctgggaggcagaggttgcagtgagccaagatcacaccactatactccagcctgggtgacagagcgagactccatcgtttctttttcgagcgaattacacagttgtcttggcagcgtgatttgccctctggttcctgctttatcagtttggtgattctttgtacagattgataaccatgaaaaagtctaaagtagggcagttccggagcagccttttcccataaagcaagcgggtacctcacaaaactccaggcaaaagaatgaatgatagagcactcaccaatagcgagtggagaagagtattttgtcgaagtttgcaaaccaatctttgggagccagaggtgggaattttaaaatgaggtcttttccttggaattttcttaaagtggtatcgttgcctgttgatattgaagtttgtcaaagaacgtgaaatcaccagcttagaggatttttttccccccttcaagacgctaagcaaaagccactccgtcgacatcaaaccccacgccggagccggaagcaagagtaga

SEQ ID NO: 18288 - RNA, 532 nt, Homo sapiens
  source 1..532: mol_type = other RNA
tgaagtaccagctactcgagaggctgaggcaggagaatcgcttgaacctgggaggcagaggttgcagtgagccaagatcacaccactatactccagcctgggtgacagagcgagactccatctttcaaaaatccactgataatctgggcatgatgctttcaaacttcaccctaaagagaaaaatgctctctgaacactcttcttcctgctgtctttaaattgtgcctgtattttctctgcttttcctttgacactcaatcactcctttaaaacttgtaaaaaaccggaaaagtttctgtaactctccaatctccaactatgtcgtaaaatcccttgccagtttacccagtctgctggagaggctcaccgtttctttttcgagcgaattacacagttgtcttggcagcgtgatttgccctctggttcctgctttatcagtttggtgattctttgtacagattgataaccatgaaaaagtctaaagtagggcagttccggagcagccttttcccataaagcaagcgggtacctc

SEQ ID NO: 18289 - RNA, 558 nt, Homo sapiens
  source 1..558: mol_type = other RNA
tgaagtaccagctactcgagaggctgaggcaggagaatcgcttgaacctgggaggcagaggttgcagtgagccaagatcacaccactatactccagcctgggtgacagagcgagactccatctttcaaaaatccactgataatctgggcatgatgctttcaaacttcaccctaaagagaaaaatgctctctgaacactcttcttcctgctgtctttaaattgtgcctgtattttctctgcttttcctttgacactcaatcactcctttaaaacttgtaaaaaaccggaaaagtttctgtaactctccaatctccaactatgtcgtaaaatcccttgccagtttacccagtctgctggagaggctcaccgtttctttttcgagcgaattacacagttgtcttggcagcgtgatttgccctctggttcctgctttatcagtttggtgattctttgtacagattgataaccatgaaaaagtctaaagtagggcagttccggagcagccttttcccataaagcaagcgggtacctcacaaaactccaggcaaaagaatgaat

SEQ ID NO: 18290 - RNA, 570 nt, Homo sapiens
  source 1..570: mol_type = other RNA
tgaagtaccagctactcgagaggctgaggcaggagaatcgcttgaacctgggaggcagaggttgcagtgagccaagatcacaccactatactccagcctgggtgacagagcgagactccatctttcaaaaatccactgataatctgggcatgatgctttcaaacttcaccctaaagagaaaaatgctctctgaacactcttcttcctgctgtctttaaattgtgcctgtattttctctgcttttcctttgacactcaatcactcctttaaaacttgtaaaaaaccggaaaagtttctgtaactctccaatctccaactatgtcgtaaaatcccttgccagtttacccagtctgctggagaggctcaccgtttctttttcgagcgaattacacagttgtcttggcagcgtgatttgccctctggttcctgctttatcagtttggtgattctttgtacagattgataaccatgaaaaagtctaaagtagggcagttccggagcagccttttcccataaagcaagcgggtacctcacaaaactccaggcaaaagaatgaatgatagagcactc

SEQ ID NO: 18291 - RNA, 821 nt, Homo sapiens
  source 1..821: mol_type = other RNA
tgaagtaccagctactcgagaggctgaggcaggagaatcgcttgaacctgggaggcagaggttgcagtgagccaagatcacaccactatactccagcctgggtgacagagcgagactccatctttcaaaaatccactgataatctgggcatgatgctttcaaacttcaccctaaagagaaaaatgctctctgaacactcttcttcctgctgtctttaaattgtgcctgtattttctctgcttttcctttgacactcaatcactcctttaaaacttgtaaaaaaccggaaaagtttctgtaactctccaatctccaactatgtcgtaaaatcccttgccagtttacccagtctgctggagaggctcaccgtttctttttcgagcgaattacacagttgtcttggcagcgtgatttgccctctggttcctgctttatcagtttggtgattctttgtacagattgataaccatgaaaaagtctaaagtagggcagttccggagcagccttttcccataaagcaagcgggtacctcacaaaactccaggcaaaagaatgaatgatagagcactcaccaatagcgagtggagaagagtattttgtcgaagtttgcaaaccaatctttgggagccagaggtgggaattttaaaatgaggtcttttccttggaattttcttaaagtggtatcgttgcctgttgatattgaagtttgtcaaagaacgtgaaatcaccagcttagaggatttttttccccccttcaagacgctaagcaaaagccactccgtcgacatcaaaccccacgccggagccggaagcaagagtag

SEQ ID NO: 18292 - RNA, 2389 nt, Homo sapiens
  source 1..2389: mol_type = other RNA
tgaagtaccagctactcgagaggctgaggcaggagaatcgcttgagcccgggaggcaggggttgcagtgagcaaagattgcgccattgcacccccagcctgggcaacaagagtgaaactccatctcaaaaaataaaataaaataaaaataaataaataaaaatgctagggaaacaaaggtatatccccagtctctgcctctattaagcccacctcttgtctgttccagggtgaaagagtgagctttacacgttatgctggcttatatttcccaaacatttccccaacacgatgcaggcatattacatggctcaggacagtaataagatggattaagcattctgtacaacttaaaaagcattatcaaaccccttcaaaaacaaactaaacaatggctggttggatacctgtgaatgacccaaggctttctaagataaactatttagaactcaatagaggggtctcctaatgaaatcaagccttctggaaaggaaacaacttgtagtttgcaagaactcaaagatactttggatccactacagagcttgccaaaattatgaaatgaaattttttactaagcagacaaaggaagatgcattatatttaaaaatcactgtcaattttactaggatttagaatataaaacctttacatctcttttacaataaagagaatttagagctcacttgtcacgaaaatatttttcattattaaaaaaaattgttataaagttatttcttctgatatggagtttcaaagcatctaacataaccgcttcagaatctccacagtgcaaaaataaacaacatgcatacacttaagaactttacattctttgaaaaacaatacaaattggaaagaaaattagtatgtgatcaaagagagtcagagctcaagtctgaactttgccaataaaggcagatgatctgaagagttattttcgtttggaagtccattaacagtccataagtcttgttctgtaagaagtgacagtctagctagaagtttcaagccaccaaccaaagcaacttcagctcctgggtgcccagcaacatcttccttttctgcagagtagaaaatataatccacagttatggcacttcgggaatgacaggtggtcacttctggaattccagtgtcaggaaagtaatgtgaataaacagatgacaaactgaaatggtgctgtaaatttgaagacaatttttcagctgtcactaggacctctgtttgcttcagctgtgtttgtgtcagatcactgtctgtcttttctacttttggtacctgctgtacctcatacacacagttctgtgagatacctaggtttgggggccaaattggaatagataaaattctttgtccccgtgaagactgttcctggccagatacctttcctatgggaagtccttcataattcaattttccttcctttatgaaactatatagtggagaaccaggaacagaattaaagtcaccacacataacaatagggcagaagctgccatctttctggtgggcaacactggaaatctctgccagtagcattgccaattgcgtcagcttaatatcacctcgccttggattatacaacagatgcgtatttgctacgcagattgcagggcaggcagcatatggaattttgggctgtaagagtaaaactaatccaacattgtctctgtccaacagagaaatatcagggcggaagaattccactgggttcactgacaagagtgaaaatttggaatgtttgaagcaaatagcacagccatcaggtttccttcctgtccgcatcttatattcacagtgataacccagtgattccaaacttggcctgatctctgctccataatgatcttcttgaacttcttgcaaacaaagtacgtctgcatcaaaatgtttaatttctttcagaatattgggaaacctaaaactccagtgtaatactggccgccggcaatgtctataaaggtgagagttatcttccagtaaatcttgtgaaagtatattataggacatcactgaaaagtcaaacttgttctcactgtcttcacatttgggatcaacatttttgtctcctaggatcttcgttttttctttatcatggctacatatatattcccaattccgctttatcacaccggcctcttcccaccacacagtggccgtagcccttcctcacacagcgccaggcttccatcttcgccctccgcgtgcgtccagttcccaggccccgggttccacctcaatctctataatcgatgcgacggcctaaagtatctagggaaccccatcactcttaagtaccgactccagtcctggctgcaaggcatgctgggaggtgcagtctcgccggccggcctacactccatcttgcgcagtcagagtccctgaat

SEQ ID NO: 18293 - RNA, 2744 nt, Homo sapiens
  source 1..2744: mol_type = other RNA
tgaagtaccagctactcgagaggctgaggcaggagaatcgcttgagcccgggaggcaggggttgcagtgagcaaagattgcgccattgcacccccagcctgggcaacaagagtgaaactccatctcaaaaaataaaataaaataaaaataaataaataaaaatgctagggaaacaaaggtatatccccagtctctgcctctattaagcccacctcttgtctgttccagggtgaaagagtgagctttacacgttatgctggcttatatttcccaaacatttccccaacacgatgcaggcatattacatggctcaggacagtaataagatggattaagcattctgtacaacttaaaaagcattatcaaaccccttcaaaaacaaactaaacaatggctggttggatacctgtgaatgacccaaggctttctaagataaactatttagaactcaatagaggggtctcctaatgaaatcaagccttctggaaaggaaacaacttgtagtttgcaagaactcaaagatactttggatccactacagagcttgccaaaattatgaaatgaaattttttactaagcagacaaaggaagatgcattatatttaaaaatcactgtcaattttactaggatttagaatataaaacctttacatctcttttacaataaagagaatttagagctcacttgtcacgaaaatatttttcattattaaaaaaaattgttataaagttatttcttctgatatggagtttcaaagcatctaacataaccgcttcagaatctccacagtgcaaaaataaacaacatgcatacacttaagaactttacattctttgaaaaacaatacaaattggaaagaaaattagtatgtgatcaaagagagtcagagctcaagtctgaactttgccaataaaggcagatgatctgaagagttattttcgtttggaagtccattaacagtccataagtcttgttctgtaagaagtgacagtctagctagaagtttcaagccaccaaccaaagcaacttcagctcctgggtgcccagcaacatcttccttttctgcagagtagaaaatataatccacagttatggcacttcgggaatgacaggtggtcacttctggaattccagtgtcaggaaagtaatgtgaataaacagatgacaaactgaaatggtgctgtaaatttgaagacaatttttcagctgtcactaggacctctgtttgcttcagctgtgtttgtgtcagatcactgtctgtcttttctacttttggtacctgctgtacctcatacacacagttctgtgagatacctaggtttgggggccaaattggaatagataaaattctttgtccccgtgaagactgttcctggccagatacctttcctatgggaagtccttcataattcaattttccttcctttatgaaactatatagtggagaaccaggaacagaattaaagtcaccacacataacaatagggcagaagctgccatctttctggtgggcaacactggaaatctctgccagtagcattgccaattgcgtcagcttaatatcacctcgccttggattatacaacagatgcgtatttgctacgcagattgcagggcaggcagcatatggaattttgggctgtaagagtaaaactaatccaacattgtctctgtccaacagagaaatatcagggcggaagaattccactgggttcactgacaagagtgaaaatttggaatgtttgaagcaaatagcacagccatcaggtttccttcctgtccgcatcttatattcacagtgataacccagtgattccaaacttggcctgatctctgctccataatgatcttcttgaacttcttgcaaacaaagtacgtctgcatcaaaatgtttaatttctttcagaatattgggaaacctaaaactccagtgtaatactggccgccggcaatgtctataaaggtgagagttatcttccagtaaatcttgtgaaagtatattataggacatcactgaaaagtcaaacttgttctcactgtcttcacatttgggatcaacatttttgtctcctaggatcttcgttttttctttatcatggctacatatatattcccaattccgctttatcacaccttccatatcaggaggaacaaggtgatcacagcagagaagacagatgaatcaaagaaagtaagcaataggcctgatcaggtttttagggtgcctaattacaaagtcataattgtatcacacaaatccttcaaataccactttaaagtgataggcaagttagcaatgctgttttcttgattgaaaagtattagtgaaatatcggaagtcacaaatatggcttaacgaagagcattttccttattcacaacacacatcaacaaaaatcaagcccctcctgggcgtgtgccacacacgcgcctccaagggatcaggcccgccgagacctactgcggagaggcggcctccccgccgacgctcggttcccgggacggtgctgcggagtgtgtggagcaggccagcgctggtctggaggctgggttgggggaagcaggccagggatccaaagccactggcacaagcctggccggcggcccatgaactccgcgccaagaccccagacctcgttggcccagcgtcccgccagctgcgcggcgggtttacctatcccgcttggtctctggaggctcgtcccggatgcaccatcgcccagaccctcttcctcttccttcc

SEQ ID NO: 18294 - RNA, 2640 nt, Homo sapiens
  source 1..2640: mol_type = other RNA
tgaagtaccagctactcgagaggctgaggcaggagaatcgcttgagcccgggaggcaggggttgcagtgagcaaagattgcgccattgcacccccagcctgggcaacaagagtgaaactccatctcaaaaaataaaataaaataaaaataaataaataaaaatgctagggaaacaaaggtatatccccagtctctgcctctattaagcccacctcttgtctgttccagggtgaaagagtgagctttacacgttatgctggcttatatttcccaaacatttccccaacacgatgcaggcatattacatggctcaggacagtaataagatggattaagcattctgtacaacttaaaaagcattatcaaaccccttcaaaaacaaactaaacaatggctggttggatacctgtgaatgacccaaggctttctaagataaactatttagaactcaatagaggggtctcctaatgaaatcaagccttctggaaaggaaacaacttgtagtttgcaagaactcaaagatactttggatccactacagagcttgccaaaattatgaaatgaaattttttactaagcagacaaaggaagatgcattatatttaaaaatcactgtcaattttactaggatttagaatataaaacctttacatctcttttacaataaagagaatttagagctcacttgtcacgaaaatatttttcattattaaaaaaaattgttataaagttatttcttctgatatggagtttcaaagcatctaacataaccgcttcagaatctccacagtgcaaaaataaacaacatgcatacacttaagaactttacattctttgaaaaacaatacaaattggaaagaaaattagtatgtgatcaaagagagtcagagctcaagtctgaactttgccaataaaggcagatgatctgaagagttattttcgtttggaagtccattaacagtccataagtcttgttctgtaagaagtgacagtctagctagaagtttcaagccaccaaccaaagcaacttcagctcctgggtgcccagcaacatcttccttttctgcagagtagaaaatataatccacagttatggcacttcgggaatgacaggtggtcacttctggaattccagtgtcaggaaagtaatgtgaataaacagatgacaaactgaaatggtgctgtaaatttgaagacaatttttcagctgtcactaggacctctgtttgcttcagctgtgtttgtgtcagatcactgtctgtcttttctacttttggtacctgctgtacctcatacacacagttctgtgagatacctaggtttgggggccaaattggaatagataaaattctttgtccccgtgaagactgttcctggccagatacctttcctatgggaagtccttcataattcaattttccttcctttatgaaactatatagtggagaaccaggaacagaattaaagtcaccacacataacaatagggcagaagctgccatctttctggtgggcaacactggaaatctctgccagtagcattgccaattgcgtcagcttaatatcacctcgccttggattatacaacagatgcgtatttgctacgcagattgcagggcaggcagcatatggaattttgggctgtaagagtaaaactaatccaacattgtctctgtccaacagagaaatatcagggcggaagaattccactgggttcactgacaagagtgaaaatttggaatgtttgaagcaaatagcacagccatcaggtttccttcctgtccgcatcttatattcacagtgataacccagtgattccaaacttggcctgatctctgctccataatgatcttcttgaacttcttgcaaacaaagtacgtctgcatcaaaatgtttaatttctttcagaatattgggaaacctaaaactccagtgtaatactggccgccggcaatgtctataaaggtgagagttatcttccagtaaatcttgtgaaagtatattataggacatcactgaaaagtcaaacttgttctcactgtcttcacatttgggatcaacatttttgtctcctaggatcttcgttttttctttatcatggctacatatatattcccaattccgctttatcacaccttccatatcaggaggaacaaggtgatcacagcagagaagacagatgaatcaaagaaagtaagcaataggcctgatcaggtttttagggtgcctaattacaaagtcataattgtatcacacaaatccttcaaataccactttaaagtgataggcaagttagcaatgctgttttcttgattgaaaagtattagtgaaatatcggaagtcacaaatatggcttaacgaagagcattttccttattcacaacaccggcctcttcccaccacacagtggccgtagcccttcctcacacagcgccaggcttccatcttcgccctccgcgtgcgtccagttcccaggccccgggttccacctcaatctctataatcgatgcgacggcctaaagtatctagggaaccccatcactcttaagtaccgactccagtcctggctgcaaggcatgctgggaggtgcagtctcgccggccggcctacactccatcttgcgcagtcagagtccctgaat

SEQ ID NO: 18295 - RNA, 3041 nt, Homo sapiens
  source 1..3041: mol_type = other RNA
tgaagtaccagctactcgagaggctgaggcaggagaatcgcttgagcccgggaggcaggggttgcagtgagcaaagattgcgccattgcacccccagcctgggcaacaagagtgaaactccatctcaaaaaataaaataaaataaaaataaataaataaaaatgctagggaaacaaaggtatatccccagtctctgcctctattaagcccacctcttgtctgttccagggtgaaagagtgagctttacacgttatgctggcttatatttcccaaacatttccccaacacgatgcaggcatattacatggctcaggacagtaataagatggattaagcattctgtacaacttaaaaagcattatcaaaccccttcaaaaacaaactaaacaatggctggttggatacctgtgaatgacccaaggctttctaagataaactatttagaactcaatagaggggtctcctaatgaaatcaagccttctggaaaggaaacaacttgtagtttgcaagaactcaaagatactttggatccactacagagcttgccaaaattatgaaatgaaattttttactaagcagacaaaggaagatgcattatatttaaaaatcactgtcaattttactaggatttagaatataaaacctttacatctcttttacaataaagagaatttagagctcacttgtcacgaaaatatttttcattattaaaaaaaattgttataaagttatttcttctgatatggagtttcaaagcatctaacataaccgcttcagaatctccacagtgcaaaaataaacaacatgcatacacttaagaactttacattctttgaaaaacaatacaaattggaaagaaaattagtatgtgatcaaagagagtcagagctcaagtctgaactttgccaataaaggcagatgatctgaagagttattttcgtttggaagtccattaacagtccataagtcttgttctgtaagaagtgacagtctagctagaagtttcaagccaccaaccaaagcaacttcagctcctgggtgcccagcaacatcttccttttctgcagagtagaaaatataatccacagttatggcacttcgggaatgacaggtggtcacttctggaattccagtgtcaggaaagtaatgtgaataaacagatgacaaactgaaatggtgctgtaaatttgaagacaatttttcagctgtcactaggacctctgtttgcttcagctgtgtttgtgtcagatcactgtctgtcttttctacttttggtacctgctgtacctcatacacacagttctgtgagatacctaggtttgggggccaaattggaatagataaaattctttgtccccgtgaagactgttcctggccagatacctttcctatgggaagtccttcataattcaattttccttcctttatgaaactatatagtggagaaccaggaacagaattaaagtcaccacacataacaatagggcagaagctgccatctttctggtgggcaacactggaaatctctgccagtagcattgccaattgcgtcagcttaatatcacctcgccttggattatacaacagatgcgtatttgctacgcagattgcagggcaggcagcatatggaattttgggctgtaagagtaaaactaatccaacattgtctctgtccaacagagaaatatcagggcggaagaattccactgggttcactgacaagagtgaaaatttggaatgtttgaagcaaatagcacagccatcaggtttccttcctgtccgcatcttatattcacagtgataacccagtgattccaaacttggcctgatctctgctccataatgatcttcttgaacttcttgcaaacaaagtacgtctgcatcaaaatgtttaatttctttcagaatattgggaaacctaaaactccagtgtaatactggccgccggcaatgtctataaaggtgagagttatcttccagtaaatcttgtgaaagtatattataggacatcactgaaaagtcaaacttgttctcactgtcttcacatttgggatcaacatttttgtctcctaggatcttcgttttttctttatcatggctacatatatattcccaattccgctttatcacaccttccatatcaggaggaacaaggtgatcacagcagagaagacagatgaatcaaagaaagtaagcaataggcctgatcaggtttttagggtgcctaattacaaagtcataattgtatcacacaaatccttcaaataccactttaaagtgataggcaagttagcaatgctgttttcttgattgaaaagtattagtgaaatatcggaagtcacaaatatggcttaacgaagagcattttccttattcacaacaccttggtgttttcttcgttttgatgaaggctcatctccctcagcgttcatgacgtaactagagagatgaatcaaagatgtctggctcaggttgtcaggtctccagttacagtactggaactgagttctagactcaaacaaacagggtggtctccaatttagtgaaaaatgcctactactgaagtatgggtaaggagctcgagagtaatgtccaggccacctcatacaactagaaatatgtctgttccagcaacacctttgcagattctcccacggtgtagtccagtctctgcccagactcctcgagtgatggggaaacatggggtatacatcaacaaaaatcaagcccctcctgggcgtgtgccacacacgcgcctccaagggatcaggcccgccgagacctactgcggagaggcggcctccccgccgacgctcggttcccgggacggtgctgcggagtgtgtggagcaggccagcgctggtctggaggctgggttgggggaagcaggccagggatccaaagccactggcacaagcctggccggcggcccatgaactccgcgccaagaccccagacctcgttggcccagcgtcccgccagctgcgcggcgggtttacctatcccgcttggtctctggaggctcgtcccggatgcacc

SEQ ID NO: 18296 - RNA, 2971 nt, Homo sapiens
  source 1..2971: mol_type = other RNA
tgaagtaccagctactcgagaggctgaggcaggagaatcgcttgagcccgggaggcaggggttgcagtgagcaaagattgcgccattgcacccccagcctgggcaacaagagtgaaactccatctcaaaaaataaaataaaataaaaataaataaataaaaatgctagggaaacaaaggtatatccccagtctctgcctctattaagcccacctcttgtctgttccagggtgaaagagtgagctttacacgttatgctggcttatatttcccaaacatttccccaacacgatgcaggcatattacatggctcaggacagtaataagatggattaagcattctgtacaacttaaaaagcattatcaaaccccttcaaaaacaaactaaacaatggctggttggatacctgtgaatgacccaaggctttctaagataaactatttagaactcaatagaggggtctcctaatgaaatcaagccttctggaaaggaaacaacttgtagtttgcaagaactcaaagatactttggatccactacagagcttgccaaaattatgaaatgaaattttttactaagcagacaaaggaagatgcattatatttaaaaatcactgtcaattttactaggatttagaatataaaacctttacatctcttttacaataaagagaatttagagctcacttgtcacgaaaatatttttcattattaaaaaaaattgttataaagttatttcttctgatatggagtttcaaagcatctaacataaccgcttcagaatctccacagtgcaaaaataaacaacatgcatacacttaagaactttacattctttgaaaaacaatacaaattggaaagaaaattagtatgtgatcaaagagagtcagagctcaagtctgaactttgccaataaaggcagatgatctgaagagttattttcgtttggaagtccattaacagtccataagtcttgttctgtaagaagtgacagtctagctagaagtttcaagccaccaaccaaagcaacttcagctcctgggtgcccagcaacatcttccttttctgcagagtagaaaatataatccacagttatggcacttcgggaatgacaggtggtcacttctggaattccagtgtcaggaaagtaatgtgaataaacagatgacaaactgaaatggtgctgtaaatttgaagacaatttttcagctgtcactaggacctctgtttgcttcagctgtgtttgtgtcagatcactgtctgtcttttctacttttggtacctgctgtacctcatacacacagttctgtgagatacctaggtttgggggccaaattggaatagataaaattctttgtccccgtgaagactgttcctggccagatacctttcctatgggaagtccttcataattcaattttccttcctttatgaaactatatagtggagaaccaggaacagaattaaagtcaccacacataacaatagggcagaagctgccatctttctggtgggcaacactggaaatctctgccagtagcattgccaattgcgtcagcttaatatcacctcgccttggattatacaacagatgcgtatttgctacgcagattgcagggcaggcagcatatggaattttgggctgtaagagtaaaactaatccaacattgtctctgtccaacagagaaatatcagggcggaagaattccactgggttcactgacaagagtgaaaatttggaatgtttgaagcaaatagcacagccatcaggtttccttcctgtccgcatcttatattcacagtgataacccagtgattccaaacttggcctgatctctgctccataatgatcttcttgaacttcttgcaaacaaagtacgtctgcatcaaaatgtttaatttctttcagaatattgggaaacctaaaactccagtgtaatactggccgccggcaatgtctataaaggtgagagttatcttccagtaaatcttgtgaaagtatattataggacatcactgaaaagtcaaacttgttctcactgtcttcacatttgggatcaacatttttgtctcctaggatcttcgttttttctttatcatggctacatatatattcccaattccgctttatcacaccttccatatcaggaggaacaaggtgatcacagcagagaagacagatgaatcaaagaaagtaagcaataggcctgatcaggtttttagggtgcctaattacaaagtcataattgtatcacacaaatccttcaaataccactttaaagtgataggcaagttagcaatgctgttttcttgattgaaaagtattagtgaaatatcggaagtcacaaatatggcttaacgaagagcattttccttattcacaacaccttggtgttttcttcgttttgatgaaggctcatctccctcagcgttcatgacgtaactagagagatgaatcaaagatgtctggctcaggttgtcaggtctccagttacagtactggaactgagttctagactcaaacaaacagggtggtctccaatttagtgaaaaatgcctactactgaagtatgggtaaggagctcgagagtaatgtccaggccacctcatacaactagaaatatgtctgttccagcaacacctttgcagattctcccacggtgtagtccagtctctgcccagactcctcgagtgatggggaaacatggggtatcggcctcttcccaccacacagtggccgtagcccttcctcacacagcgccaggcttccatcttcgccctccgcgtgcgtccagttcccaggccccgggttccacctcaatctctataatcgatgcgacggcctaaagtatctagggaaccccatcactcttaagtaccgactccagtcctggctgcaaggcatgctgggaggtgcagtctcgccggccggcctacactccatcttgcgcagtcagagtccctgaatgcctt

SEQ ID NO: 18297 - RNA, 2784 nt, Homo sapiens
  source 1..2784: mol_type = other RNA
tgaagtaccagctactcgagaggctgaggcaggagaatcgcttgagcccgggaggcaggggttgcagtgagcaaagattgcgccattgcacccccagcctgggcaacaagagtgaaactccatctcaaaaaataaaataaaataaaaataaataaataaaaatgctagggaaacaaaggtatatccccagtctctgcctctattaagcccacctcttgtctgttccagggtgaaagagtgagctttacacgttatgctggcttatatttcccaaacatttccccaacacgatgcaggcatattacatggctcaggacagtaataagatggattaagcattctgtacaacttaaaaagcattatcaaaccccttcaaaaacaaactaaacaatggctggttggatacctgtgaatgacccaaggctttctaagataaactatttagaactcaatagaggggtctcctaatgaaatcaagccttctggaaaggaaacaacttgtagtttgcaagaactcaaagatactttggatccactacagagcttgccaaaattatgaaatgaaattttttactaagcagacaaaggaagatgcattatatttaaaaatcactgtcaattttactaggatttagaatataaaacctttacatctcttttacaataaagagaatttagagctcacttgtcacgaaaatatttttcattattaaaaaaaattgttataaagttatttcttctgatatggagtttcaaagcatctaacataaccgcttcagaatctccacagtgcaaaaataaacaacatgcatacacttaagaactttacattctttgaaaaacaatacaaattggaaagaaaattagtatgtgatcaaagagagtcagagctcaagtctgaactttgccaataaaggcagatgatctgaagagttattttcgtttggaagtccattaacagtccataagtcttgttctgtaagaagtgacagtctagctagaagtttcaagccaccaaccaaagcaacttcagctcctgggtgcccagcaacatcttccttttctgcagagtagaaaatataatccacagttatggcacttcgggaatgacaggtggtcacttctggaattccagtgtcaggaaagtaatgtgaataaacagatgacaaactgaaatggtgctgtaaatttgaagacaatttttcagctgtcactaggacctctgtttgcttcagctgtgtttgtgtcagatcactgtctgtcttttctacttttggtacctgctgtacctcatacacacagttctgtgagatacctaggtttgggggccaaattggaatagataaaattctttgtccccgtgaagactgttcctggccagatacctttcctatgggaagtccttcataattcaattttccttcctttatgaaactatatagtggagaaccaggaacagaattaaagtcaccacacataacaatagggcagaagctgccatctttctggtgggcaacactggaaatctctgccagtagcattgccaattgcgtcagcttaatatcacctcgccttggattatacaacagatgcgtatttgctacgcagattgcagggcaggcagcatatggaattttgggctgtaagagtaaaactaatccaacattgtctctgtccaacagagaaatatcagggcggaagaattccactgggttcactgacaagagtgaaaatttggaatgtttgaagcaaatagcacagccatcaggtttccttcctgtccgcatcttatattcacagtgataacccagtgattccaaacttggcctgatctctgctccataatgatcttcttgaacttcttgcaaacaaagtacgtctgcatcaaaatgtttaatttctttcagaatattgggaaacctaaaactccagtgtaatactggccgccggcaatgtctataaaggtgagagttatcttccagtaaatcttgtgaaagtatattataggacatcactgaaaagtcaaacttgttctcactgtcttcacatttgggatcaacatttttgtctcctaggatcttcgttttttctttatcatggctacatatatattcccaattccgctttatcacaccttccatatcaggaggaacaaggtgatcacagcagagaagacagatgaatcaaagaaagtaagcaataggcctgatcaggtttttagggtgcctaattacaaagtcataattgtatcacacaaatccttcaaataccactttaaagtgataggcaagttagcaatgctgttttcttgattgaaaagtattagtgaaatatcggaagtcacaaatatggcttaacgaagagcattttccttattcacaacaccttggtgttttcttcgttttgatgaaggctcatctccctcagcgttcatgacgtaactagagagatgaatcaaagatgtctggctcaggttgtcaggtctccagttacagtactggaactgagttctagactcaaacaaacagggtggtctccaatttagtgaaaaatgcctactactgaagtatgggtaaggagctcgagagtaatgtccaggccacctcatacaactagaaatatgtctgttccagcaacacctttgcagattctcccacggtgtagtccagtctctgcccagactcctcgagtgatggggaaacatggggtatctatcccgcttggtctctggaggctcgtcccggatgcaccatcgcccagaccctcttcctcttccttccaccc

SEQ ID NO: 18298 - RNA, 2995 nt, Homo sapiens
  source 1..2995: mol_type = other RNA
tgaagtaccagctactcgagaggctgaggcaggagaatcgcttgagcccgggaggcaggggttgcagtgagcaaagattgcgccattgcacccccagcctgggcaacaagagtgaaactccatctcaaaaaataaaataaaataaaaataaataaataaaaatgctagggaaacaaaggtatatccccagtctctgcctctattaagcccacctcttgtctgttccagggtgaaagagtgagctttacacgttatgctggcttatatttcccaaacatttccccaacacgatgcaggcatattacatggctcaggacagtaataagatggattaagcattctgtacaacttaaaaagcattatcaaaccccttcaaaaacaaactaaacaatggctggttggatacctgtgaatgacccaaggctttctaagataaactatttagaactcaatagaggggtctcctaatgaaatcaagccttctggaaaggaaacaacttgtagtttgcaagaactcaaagatactttggatccactacagagcttgccaaaattatgaaatgaaattttttactaagcagacaaaggaagatgcattatatttaaaaatcactgtcaattttactaggatttagaatataaaacctttacatctcttttacaataaagagaatttagagctcacttgtcacgaaaatatttttcattattaaaaaaaattgttataaagttatttcttctgatatggagtttcaaagcatctaacataaccgcttcagaatctccacagtgcaaaaataaacaacatgcatacacttaagaactttacattctttgaaaaacaatacaaattggaaagaaaattagtatgtgatcaaagagagtcagagctcaagtctgaactttgccaataaaggcagatgatctgaagagttattttcgtttggaagtccattaacagtccataagtcttgttctgtaagaagtgacagtctagctagaagtttcaagccaccaaccaaagcaacttcagctcctgggtgcccagcaacatcttccttttctgcagagtagaaaatataatccacagttatggcacttcgggaatgacaggtggtcacttctggaattccagtgtcaggaaagtaatgtgaataaacagatgacaaactgaaatggtgctgtaaatttgaagacaatttttcagctgtcactaggacctctgtttgcttcagctgtgtttgtgtcagatcactgtctgtcttttctacttttggtacctgctgtacctcatacacacagttctgtgagatacctaggtttgggggccaaattggaatagataaaattctttgtccccgtgaagactgttcctggccagatacctttcctatgggaagtccttcataattcaattttccttcctttatgaaactatatagtggagaaccaggaacagaattaaagtcaccacacataacaatagggcagaagctgccatctttctggtgggcaacactggaaatctctgccagtagcattgccaattgcgtcagcttaatatcacctcgccttggattatacaacagatgcgtatttgctacgcagattgcagggcaggcagcatatggaattttgggctgtaagagtaaaactaatccaacattgtctctgtccaacagagaaatatcagggcggaagaattccactgggttcactgacaagagtgaaaatttggaatgtttgaagcaaatagcacagccatcaggtttccttcctgtccgcatcttatattcacagtgataacccagtgattccaaacttggcctgatctctgctccataatgatcttcttgaacttcttgcaaacaaagtacgtctgcatcaaaatgtttaatttctttcagaatattgggaaacctaaaactccagtgtaatactggccgccggcaatgtctataaaggtgagagttatcttccagtaaatcttgtgaaagtatattataggacatcactgaaaagtcaaacttgttctcactgtcttcacatttgggatcaacatttttgtctcctaggatcttcgttttttctttatcatggctacatatatattcccaattccgctttatcacaccttccatatcaggaggaacaaggtgatcacagcagagaagacagatgaatcaaagaaagtaagcaataggcctgatcaggtttttagggtgcctaattacaaagtcataattgtatcacacaaatccttcaaataccactttaaagtgataggcaagttagcaatgctgttttcttgattgaaaagtattagtgaaatatcggaagtcacaaatatggcttaacgaagagcattttccttattcacaacaccttggtgttttcttcgttttgatgaaggctcatctccctcagcgttcatgacgtaactagagagatgaatcaaagatgtctggctcaggttgtcaggtctccagttacagtactggaactgagttctagactcaaacaaacagggtggtctccaatttagtgaaaaatgcctactactgaagtatgggtaaggagctcgagagtaatgtccaggccacctcatacaactagaaatatgtctgttccagcaacacctttgcagattctcccacggtgtagtccagtctctgcccagactcctcgagtgatggggaaacatggggtattgcggagaggcggcctccccgccgacgctcggttcccgggacggtgctgcggagtgtgtggagcaggccagcgctggtctggaggctgggttgggggaagcaggccagggatccaaagccactggcacaagcctggccggcggcccatgaactccgcgccaagaccccagacctcgttggcccagcgtcccgccagctgcgcggcgggtttacctatcccgcttggtctctggaggctcgtcccggatgcaccatcgcccagaccctcttcctcttccttccac

SEQ ID NO: 18299 - RNA, 2672 nt, Homo sapiens
  source 1..2672: mol_type = other RNA
tgaagtaccagctactcgagaggctgaggcaggagaatcgcttgagcccgggaggcaggggttgcagtgagcaaagattgcgccattgcacccccagcctgggcaacaagagtgaaactccatctcaaaaaataaaataaaataaaaataaataaataaaaatgctagggaaacaaaggtatatccccagtctctgcctctattaagcccacctcttgtctgttccagggtgaaagagtgagctttacacgttatgctggcttatatttcccaaacatttccccaacacgatgcaggcatattacatggctcaggacagtaataagatggattaagcattctgtacaacttaaaaagcattatcaaaccccttcaaaaacaaactaaacaatggctggttggatacctgtgaatgacccaaggctttctaagataaactatttagaactcaatagaggggtctcctaatgaaatcaagccttctggaaaggaaacaacttgtagtttgcaagaactcaaagatactttggatccactacagagcttgccaaaattatgaaatgaaattttttactaagcagacaaaggaagatgcattatatttaaaaatcactgtcaattttactaggatttagaatataaaacctttacatctcttttacaataaagagaatttagagctcacttgtcacgaaaatatttttcattattaaaaaaaattgttataaagttatttcttctgatatggagtttcaaagcatctaacataaccgcttcagaatctccacagtgcaaaaataaacaacatgcatacacttaagaactttacattctttgaaaaacaatacaaattggaaagaaaattagtatgtgatcaaagagagtcagagctcaagtctgaactttgccaataaaggcagatgatctgaagagttattttcgtttggaagtccattaacagtccataagtcttgttctgtaagaagtgacagtctagctagaagtttcaagccaccaaccaaagcaacttcagctcctgggtgcccagcaacatcttccttttctgcagagtagaaaatataatccacagttatggcacttcgggaatgacaggtggtcacttctggaattccagtgtcaggaaagtaatgtgaataaacagatgacaaactgaaatggtgctgtaaatttgaagacaatttttcagctgtcactaggacctctgtttgcttcagctgtgtttgtgtcagatcactgtctgtcttttctacttttggtacctgctgtacctcatacacacagttctgtgagatacctaggtttgggggccaaattggaatagataaaattctttgtccccgtgaagactgttcctggccagatacctttcctatgggaagtccttcataattcaattttccttcctttatgaaactatatagtggagaaccaggaacagaattaaagtcaccacacataacaatagggcagaagctgccatctttctggtgggcaacactggaaatctctgccagtagcattgccaattgcgtcagcttaatatcacctcgccttggattatacaacagatgcgtatttgctacgcagattgcagggcaggcagcatatggaattttgggctgtaagagtaaaactaatccaacattgtctctgtccaacagagaaatatcagggcggaagaattccactgggttcactgacaagagtgaaaatttggaatgtttgaagcaaatagcacagccatcaggtttccttcctgtccgcatcttatattcacagtgataacccagtgattccaaacttggcctgatctctgctccataatgatcttcttgaacttcttgcaaacaaagtacgtctgcatcaaaatgtttaatttctttcagaatattgggaaacctaaaactccagtgtaatactggccgccggcaatgtctataaaggtgagagttatcttccagtaaatcttgtgaaagtatattataggacatcactgaaaagtcaaacttgttctcactgtcttcacatttgggatcaacatttttgtctcctaggatcttcgttttttctttatcatggctacatatatattcccaattccgctttatcacaccttggtgttttcttcgttttgatgaaggctcatctccctcagcgttcatgacgtaactagagagatgaatcaaagatgtctggctcaggttgtcaggtctccagttacagtactggaactgagttctagactcaaacaaacagggtggtctccaatttagtgaaaaatgcctactactgaagtatgggtaaggagctcgagagtaatgtccaggccacctcatacaactagaaatatgtctgttccagcaacacctttgcagattctcccacggtgtagtccagtctctgcccagactcctcgagtgatggggaaacatggggtatacagcgccaggcttccatcttcgccctccgcgtgcgtccagttcccaggccccgggttccacctcaatctctataatcgatgcgacggcctaaagtatctagggaaccccatcactcttaagtaccgactccagtcctggctgcaaggcatgctgggaggtgcagtctcgccggccggcctacactccatcttgcgcagtcagagtccctga

SEQ ID NO: 18300 - RNA, 2790 nt, Homo sapiens
  source 1..2790: mol_type = other RNA
tgaagtaccagctactcgagaggctgaggcaggagaatcgcttgagcccgggaggcaggggttgcagtgagcaaagattgcgccattgcacccccagcctgggcaacaagagtgaaactccatctcaaaaaataaaataaaataaaaataaataaataaaaatgctagggaaacaaaggtatatccccagtctctgcctctattaagcccacctcttgtctgttccagggtgaaagagtgagctttacacgttatgctggcttatatttcccaaacatttccccaacacgatgcaggcatattacatggctcaggacagtaataagatggattaagcattctgtacaacttaaaaagcattatcaaaccccttcaaaaacaaactaaacaatggctggttggatacctgtgaatgacccaaggctttctaagataaactatttagaactcaatagaggggtctcctaatgaaatcaagccttctggaaaggaaacaacttgtagtttgcaagaactcaaagatactttggatccactacagagcttgccaaaattatgaaatgaaattttttactaagcagacaaaggaagatgcattatatttaaaaatcactgtcaattttactaggatttagaatataaaacctttacatctcttttacaataaagagaatttagagctcacttgtcacgaaaatatttttcattattaaaaaaaattgttataaagttatttcttctgatatggagtttcaaagcatctaacataaccgcttcagaatctccacagtgcaaaaataaacaacatgcatacacttaagaactttacattctttgaaaaacaatacaaattggaaagaaaattagtatgtgatcaaagagagtcagagctcaagtctgaactttgccaataaaggcagatgatctgaagagttattttcgtttggaagtccattaacagtccataagtcttgttctgtaagaagtgacagtctagctagaagtttcaagccaccaaccaaagcaacttcagctcctgggtgcccagcaacatcttccttttctgcagagtagaaaatataatccacagttatggcacttcgggaatgacaggtggtcacttctggaattccagtgtcaggaaagtaatgtgaataaacagatgacaaactgaaatggtgctgtaaatttgaagacaatttttcagctgtcactaggacctctgtttgcttcagctgtgtttgtgtcagatcactgtctgtcttttctacttttggtacctgctgtacctcatacacacagttctgtgagatacctaggtttgggggccaaattggaatagataaaattctttgtccccgtgaagactgttcctggccagatacctttcctatgggaagtccttcataattcaattttccttcctttatgaaactatatagtggagaaccaggaacagaattaaagtcaccacacataacaatagggcagaagctgccatctttctggtgggcaacactggaaatctctgccagtagcattgccaattgcgtcagcttaatatcacctcgccttggattatacaacagatgcgtatttgctacgcagattgcagggcaggcagcatatggaattttgggctgtaagagtaaaactaatccaacattgtctctgtccaacagagaaatatcagggcggaagaattccactgggttcactgacaagagtgaaaatttggaatgtttgaagcaaatagcacagccatcaggtttccttcctgtccgcatcttatattcacagtgataacccagtgattccaaacttggcctgatctctgctccataatgatcttcttgaacttcttgcaaacaaagtacgtctgcatcaaaatgtttaatttctttcagaatattgggaaacctaaaactccagtgtaatactggccgccggcaatgtctataaaggtgagagttatcttccagtaaatcttgtgaaagtatattataggacatcactgaaaagtcaaacttgttctcactgtcttcacatttgggatcaacatttttgtctcctaggatcttcgttttttctttatcatggctacatatatattcccaattccgctttatcacaccttggtgttttcttcgttttgatgaaggctcatctccctcagcgttcatgacgtaactagagagatgaatcaaagatgtctggctcaggttgtcaggtctccagttacagtactggaactgagttctagactcaaacaaacagggtggtctccaatttagtgaaaaatgcctactactgaagtatgggtaaggagctcgagagtaatgtccaggccacctcatacaactagaaatatgtctgttccagcaacacctttgcagattctcccacggtgtagtccagtctctgcccagactcctcgagtgatggggaaacatggggtatacatcaacaaaaatcaagcccctcctgggcgtgtgccacacacgcgcctccaagggatcaggcccgccgagacctactgcggagaggcggcctccccgccgacgctcggttcccgggacggtgctgcggagtgtgtggagcaggccagcgctggtctggaggctgggttgggggaagcaggccagggatccaaagccactggcacaagcctggccggcggcccatgaactccgcgccaagaccccagacctcgttggcccagcgtcccgccagctgcgcggcgggtttacctatcccgcttggtctctggaggctcgtcccggatgcacc

SEQ ID NO: 18301 - RNA, 2715 nt, Homo sapiens
  source 1..2715: mol_type = other RNA
tgaagtaccagctactcgagaggctgaggcaggagaatcgcttgagcccgggaggcaggggttgcagtgagcaaagattgcgccattgcacccccagcctgggcaacaagagtgaaactccatctcaaaaaataaaataaaataaaaataaataaataaaaatgctagggaaacaaaggtatatccccagtctctgcctctattaagcccacctcttgtctgttccagggtgaaagagtgagctttacacgttatgctggcttatatttcccaaacatttccccaacacgatgcaggcatattacatggctcaggacagtaataagatggattaagcattctgtacaacttaaaaagcattatcaaaccccttcaaaaacaaactaaacaatggctggttggatacctgtgaatgacccaaggctttctaagataaactatttagaactcaatagaggggtctcctaatgaaatcaagccttctggaaaggaaacaacttgtagtttgcaagaactcaaagatactttggatccactacagagcttgccaaaattatgaaatgaaattttttactaagcagacaaaggaagatgcattatatttaaaaatcactgtcaattttactaggatttagaatataaaacctttacatctcttttacaataaagagaatttagagctcacttgtcacgaaaatatttttcattattaaaaaaaattgttataaagttatttcttctgatatggagtttcaaagcatctaacataaccgcttcagaatctccacagtgcaaaaataaacaacatgcatacacttaagaactttacattctttgaaaaacaatacaaattggaaagaaaattagtatgtgatcaaagagagtcagagctcaagtctgaactttgccaataaaggcagatgatctgaagagttattttcgtttggaagtccattaacagtccataagtcttgttctgtaagaagtgacagtctagctagaagtttcaagccaccaaccaaagcaacttcagctcctgggtgcccagcaacatcttccttttctgcagagtagaaaatataatccacagttatggcacttcgggaatgacaggtggtcacttctggaattccagtgtcaggaaagtaatgtgaataaacagatgacaaactgaaatggtgctgtaaatttgaagacaatttttcagctgtcactaggacctctgtttgcttcagctgtgtttgtgtcagatcactgtctgtcttttctacttttggtacctgctgtacctcatacacacagttctgtgagatacctaggtttgggggccaaattggaatagataaaattctttgtccccgtgaagactgttcctggccagatacctttcctatgggaagtccttcataattcaattttccttcctttatgaaactatatagtggagaaccaggaacagaattaaagtcaccacacataacaatagggcagaagctgccatctttctggtgggcaacactggaaatctctgccagtagcattgccaattgcgtcagcttaatatcacctcgccttggattatacaacagatgcgtatttgctacgcagattgcagggcaggcagcatatggaattttgggctgtaagagtaaaactaatccaacattgtctctgtccaacagagaaatatcagggcggaagaattccactgggttcactgacaagagtgaaaatttggaatgtttgaagcaaatagcacagccatcaggtttccttcctgtccgcatcttatattcacagtgataacccagtgattccaaacttggcctgatctctgctccataatgatcttcttgaacttcttgcaaacaaagtacgtctgcatcaaaatgtttaatttctttcagaatattgggaaacctaaaactccagtgtaatactggccgccggcaatgtctataaaggtgagagttatcttccagtaaatcttgtgaaagtatattataggacatcactgaaaagtcaaacttgttctcactgtcttcacatttgggatcaacatttttgtctcctaggatcttcgttttttctttatcatggctacatatatattcccaattccgctttatcacaccttggtgttttcttcgttttgatgaaggctcatctccctcagcgttcatgacgtaactagagagatgaatcaaagatgtctggctcaggttgtcaggtctccagttacagtactggaactgagttctagactcaaacaaacagggtggtctccaatttagtgaaaaatgcctactactgaagtatgggtaaggagctcgagagtaatgtccaggccacctcatacaactagaaatatgtctgttccagcaacacctttgcagattctcccacggtgtagtccagtctctgcccagactcctcgagtgatggggaaacatggggtatcggcctcttcccaccacacagtggccgtagcccttcctcacacagcgccaggcttccatcttcgccctccgcgtgcgtccagttcccaggccccgggttccacctcaatctctataatcgatgcgacggcctaaagtatctagggaaccccatcactcttaagtaccgactccagtcctggctgcaaggcatgctgggaggtgcagtctcgccggccggcctacactccatcttgcgcagtcagagtccctgaat

SEQ ID NO: 18302 - RNA, 2543 nt, Homo sapiens
  source 1..2543: mol_type = other RNA
tgaagtaccagctactcgagaggctgaggcaggagaatcgcttgagcccgggaggcaggggttgcagtgagcaaagattgcgccattgcacccccagcctgggcaacaagagtgaaactccatctcaaaaaataaaataaaataaaaataaataaataaaaatgctagggaaacaaaggtatatccccagtctctgcctctattaagcccacctcttgtctgttccagggtgaaagagtgagctttacacgttatgctggcttatatttcccaaacatttccccaacacgatgcaggcatattacatggctcaggacagtaataagatggattaagcattctgtacaacttaaaaagcattatcaaaccccttcaaaaacaaactaaacaatggctggttggatacctgtgaatgacccaaggctttctaagataaactatttagaactcaatagaggggtctcctaatgaaatcaagccttctggaaaggaaacaacttgtagtttgcaagaactcaaagatactttggatccactacagagcttgccaaaattatgaaatgaaattttttactaagcagacaaaggaagatgcattatatttaaaaatcactgtcaattttactaggatttagaatataaaacctttacatctcttttacaataaagagaatttagagctcacttgtcacgaaaatatttttcattattaaaaaaaattgttataaagttatttcttctgatatggagtttcaaagcatctaacataaccgcttcagaatctccacagtgcaaaaataaacaacatgcatacacttaagaactttacattctttgaaaaacaatacaaattggaaagaaaattagtatgtgatcaaagagagtcagagctcaagtctgaactttgccaataaaggcagatgatctgaagagttattttcgtttggaagtccattaacagtccataagtcttgttctgtaagaagtgacagtctagctagaagtttcaagccaccaaccaaagcaacttcagctcctgggtgcccagcaacatcttccttttctgcagagtagaaaatataatccacagttatggcacttcgggaatgacaggtggtcacttctggaattccagtgtcaggaaagtaatgtgaataaacagatgacaaactgaaatggtgctgtaaatttgaagacaatttttcagctgtcactaggacctctgtttgcttcagctgtgtttgtgtcagatcactgtctgtcttttctacttttggtacctgctgtacctcatacacacagttctgtgagatacctaggtttgggggccaaattggaatagataaaattctttgtccccgtgaagactgttcctggccagatacctttcctatgggaagtccttcataattcaattttccttcctttatgaaactatatagtggagaaccaggaacagaattaaagtcaccacacataacaatagggcagaagctgccatctttctggtgggcaacactggaaatctctgccagtagcattgccaattgcgtcagcttaatatcacctcgccttggattatacaacagatgcgtatttgctacgcagattgcagggcaggcagcatatggaattttgggctgtaagagtaaaactaatccaacattgtctctgtccaacagagaaatatcagggcggaagaattccactgggttcactgacaagagtgaaaatttggaatgtttgaagcaaatagcacagccatcaggtttccttcctgtccgcatcttatattcacagtgataacccagtgattccaaacttggcctgatctctgctccataatgatcttcttgaacttcttgcaaacaaagtacgtctgcatcaaaatgtttaatttctttcagaatattgggaaacctaaaactccagtgtaatactggccgccggcaatgtctataaaggtgagagttatcttccagtaaatcttgtgaaagtatattataggacatcactgaaaagtcaaacttgttctcactgtcttcacatttgggatcaacatttttgtctcctaggatcttcgttttttctttatcatggctacatatatattcccaattccgctttatcacaccttggtgttttcttcgttttgatgaaggctcatctccctcagcgttcatgacgtaactagagagatgaatcaaagatgtctggctcaggttgtcaggtctccagttacagtactggaactgagttctagactcaaacaaacagggtggtctccaatttagtgaaaaatgcctactactgaagtatgggtaaggagctcgagagtaatgtccaggccacctcatacaactagaaatatgtctgttccagcaacacctttgcagattctcccacggtgtagtccagtctctgcccagactcctcgagtgatggggaaacatggggtatctatcccgcttggtctctggaggctcgtcccggatgcaccatcgcccagaccctcttcctcttccttccacccctagcccgcc

SEQ ID NO: 18303 - RNA, 2744 nt, Homo sapiens
  source 1..2744: mol_type = other RNA
tgaagtaccagctactcgagaggctgaggcaggagaatcgcttgagcccgggaggcaggggttgcagtgagcaaagattgcgccattgcacccccagcctgggcaacaagagtgaaactccatctcaaaaaataaaataaaataaaaataaataaataaaaatgctagggaaacaaaggtatatccccagtctctgcctctattaagcccacctcttgtctgttccagggtgaaagagtgagctttacacgttatgctggcttatatttcccaaacatttccccaacacgatgcaggcatattacatggctcaggacagtaataagatggattaagcattctgtacaacttaaaaagcattatcaaaccccttcaaaaacaaactaaacaatggctggttggatacctgtgaatgacccaaggctttctaagataaactatttagaactcaatagaggggtctcctaatgaaatcaagccttctggaaaggaaacaacttgtagtttgcaagaactcaaagatactttggatccactacagagcttgccaaaattatgaaatgaaattttttactaagcagacaaaggaagatgcattatatttaaaaatcactgtcaattttactaggatttagaatataaaacctttacatctcttttacaataaagagaatttagagctcacttgtcacgaaaatatttttcattattaaaaaaaattgttataaagttatttcttctgatatggagtttcaaagcatctaacataaccgcttcagaatctccacagtgcaaaaataaacaacatgcatacacttaagaactttacattctttgaaaaacaatacaaattggaaagaaaattagtatgtgatcaaagagagtcagagctcaagtctgaactttgccaataaaggcagatgatctgaagagttattttcgtttggaagtccattaacagtccataagtcttgttctgtaagaagtgacagtctagctagaagtttcaagccaccaaccaaagcaacttcagctcctgggtgcccagcaacatcttccttttctgcagagtagaaaatataatccacagttatggcacttcgggaatgacaggtggtcacttctggaattccagtgtcaggaaagtaatgtgaataaacagatgacaaactgaaatggtgctgtaaatttgaagacaatttttcagctgtcactaggacctctgtttgcttcagctgtgtttgtgtcagatcactgtctgtcttttctacttttggtacctgctgtacctcatacacacagttctgtgagatacctaggtttgggggccaaattggaatagataaaattctttgtccccgtgaagactgttcctggccagatacctttcctatgggaagtccttcataattcaattttccttcctttatgaaactatatagtggagaaccaggaacagaattaaagtcaccacacataacaatagggcagaagctgccatctttctggtgggcaacactggaaatctctgccagtagcattgccaattgcgtcagcttaatatcacctcgccttggattatacaacagatgcgtatttgctacgcagattgcagggcaggcagcatatggaattttgggctgtaagagtaaaactaatccaacattgtctctgtccaacagagaaatatcagggcggaagaattccactgggttcactgacaagagtgaaaatttggaatgtttgaagcaaatagcacagccatcaggtttccttcctgtccgcatcttatattcacagtgataacccagtgattccaaacttggcctgatctctgctccataatgatcttcttgaacttcttgcaaacaaagtacgtctgcatcaaaatgtttaatttctttcagaatattgggaaacctaaaactccagtgtaatactggccgccggcaatgtctataaaggtgagagttatcttccagtaaatcttgtgaaagtatattataggacatcactgaaaagtcaaacttgttctcactgtcttcacatttgggatcaacatttttgtctcctaggatcttcgttttttctttatcatggctacatatatattcccaattccgctttatcacaccttggtgttttcttcgttttgatgaaggctcatctccctcagcgttcatgacgtaactagagagatgaatcaaagatgtctggctcaggttgtcaggtctccagttacagtactggaactgagttctagactcaaacaaacagggtggtctccaatttagtgaaaaatgcctactactgaagtatgggtaaggagctcgagagtaatgtccaggccacctcatacaactagaaatatgtctgttccagcaacacctttgcagattctcccacggtgtagtccagtctctgcccagactcctcgagtgatggggaaacatggggtattgcggagaggcggcctccccgccgacgctcggttcccgggacggtgctgcggagtgtgtggagcaggccagcgctggtctggaggctgggttgggggaagcaggccagggatccaaagccactggcacaagcctggccggcggcccatgaactccgcgccaagaccccagacctcgttggcccagcgtcccgccagctgcgcggcgggtttacctatcccgcttggtctctggaggctcgtcccggatgcaccatcgcccagaccctcttcctcttccttccac

SEQ ID NO: 18304 - RNA, 2393 nt, Homo sapiens
  source 1..2393: mol_type = other RNA
tgaagtaccagctactcgagaggctgaggcaggagaatcgcttgagcccgggaggcaggggttgcagtgagcaaagattgcgccattgcacccccagcctgggcaacaagagtgaaactccatctcaaaaaataaaataaaataaaaataaataaataaaaatgctagggaaacaaaggtatatccccagtctctgcctctattaagcccacctcttgtctgttccagggtgaaagagtgagctttacacgttatgctggcttatatttcccaaacatttccccaacacgatgcaggcatattacatggctcaggacagtaataagatggattaagcattctgtacaacttaaaaagcattatcaaaccccttcaaaaacaaactaaacaatggctggttggatacctgtgaatgacccaaggctttctaagataaactatttagaactcaatagaggggtctcctaatgaaatcaagccttctggaaaggaaacaacttgtagtttgcaagaactcaaagatactttggatccactacagagcttgccaaaattatgaaatgaaattttttactaagcagacaaaggaagatgcattatatttaaaaatcactgtcaattttactaggatttagaatataaaacctttacatctcttttacaataaagagaatttagagctcacttgtcacgaaaatatttttcattattaaaaaaaattgttataaagttatttcttctgatatggagtttcaaagcatctaacataaccgcttcagaatctccacagtgcaaaaataaacaacatgcatacacttaagaactttacattctttgaaaaacaatacaaattggaaagaaaattagtatgtgatcaaagagagtcagagctcaagtctgaactttgccaataaaggcagatgatctgaagagttattttcgtttggaagtccattaacagtccataagtcttgttctgtaagaagtgacagtctagctagaagtttcaagccaccaaccaaagcaacttcagctcctgggtgcccagcaacatcttccttttctgcagagtagaaaatataatccacagttatggcacttcgggaatgacaggtggtcacttctggaattccagtgtcaggaaagtaatgtgaataaacagatgacaaactgaaatggtgctgtaaatttgaagacaatttttcagctgtcactaggacctctgtttgcttcagctgtgtttgtgtcagatcactgtctgtcttttctacttttggtacctgctgtacctcatacacacagttctgtgagatacctaggtttgggggccaaattggaatagataaaattctttgtccccgtgaagactgttcctggccagatacctttcctatgggaagtccttcataattcaattttccttcctttatgaaactatatagtggagaaccaggaacagaattaaagtcaccacacataacaatagggcagaagctgccatctttctggtgggcaacactggaaatctctgccagtagcattgccaattgcgtcagcttaatatcacctcgccttggattatacaacagatgcgtatttgctacgcagattgcagggcaggcagcatatggaattttgggctgtaagagtaaaactaatccaacattgtctctgtccaacagagaaatatcagggcggaagaattccactgggttcactgacaagagtgaaaatttggaatgtttgaagcaaatagcacagccatcaggtttccttcctgtccgcatcttatattcacagtgataacccagtgattccaaacttggcctgatctctgctccataatgatcttcttgaacttcttgcaaacaaagtacgtctgcatcaaaatgtttaatttctttcagaatattgggaaacctaaaactccagtgtaatactggccgccggcaatgtctataaaggtgagagttatcttccagtaaatcttgtgaaagtatattataggacatcactgaaaagtcaaacttgttctcactgtcttcacatttgggatcaacatttttgtctcctaggatcttcgttttttctttatcatggctacatatatattcccaattccgctttatcacactgaccggcctcttcccaccacacagtggccgtagcccttcctcacacagcgccaggcttccatcttcgccctccgcgtgcgtccagttcccaggccccgggttccacctcaatctctataatcgatgcgacggcctaaagtatctagggaaccccatcactcttaagtaccgactccagtcctggctgcaaggcatgctgggaggtgcagtctcgccggccggcctacactccatcttgcgcagtcagagtccctgaat

SEQ ID NO: 18305 - RNA, 2415 nt, Homo sapiens
  source 1..2415: mol_type = other RNA
tgaagtaccagctactcgagaggctgaggcaggagaatcgcttgagcccgggaggcaggggttgcagtgagcaaagattgcgccattgcacccccagcctgggcaacaagagtgaaactccatctcaaaaaataaaataaaataaaaataaataaataaaaatgctagggaaacaaaggtatatccccagtctctgcctctattaagcccacctcttgtctgttccagggtgaaagagtgagctttacacgttatgctggcttatatttcccaaacatttccccaacacgatgcaggcatattacatggctcaggacagtaataagatggattaagcattctgtacaacttaaaaagcattatcaaaccccttcaaaaacaaactaaacaatggctggttggatacctgtgaatgacccaaggctttctaagataaactatttagaactcaatagaggggtctcctaatgaaatcaagccttctggaaaggaaacaacttgtagtttgcaagaactcaaagatactttggatccactacagagcttgccaaaattatgaaatgaaattttttactaagcagacaaaggaagatgcattatatttaaaaatcactgtcaattttactaggatttagaatataaaacctttacatctcttttacaataaagagaatttagagctcacttgtcacgaaaatatttttcattattaaaaaaaattgttataaagttatttcttctgatatggagtttcaaagcatctaacataaccgcttcagaatctccacagtgcaaaaataaacaacatgcatacacttaagaactttacattctttgaaaaacaatacaaattggaaagaaaattagtatgtgatcaaagagagtcagagctcaagtctgaactttgccaataaaggcagatgatctgaagagttattttcgtttggaagtccattaacagtccataagtcttgttctgtaagaagtgacagtctagctagaagtttcaagccaccaaccaaagcaacttcagctcctgggtgcccagcaacatcttccttttctgcagagtagaaaatataatccacagttatggcacttcgggaatgacaggtggtcacttctggaattccagtgtcaggaaagtaatgtgaataaacagatgacaaactgaaatggtgctgtaaatttgaagacaatttttcagctgtcactaggacctctgtttgcttcagctgtgtttgtgtcagatcactgtctgtcttttctacttttggtacctgctgtacctcatacacacagttctgtgagatacctaggtttgggggccaaattggaatagataaaattctttgtccccgtgaagactgttcctggccagatacctttcctatgggaagtccttcataattcaattttccttcctttatgaaactatatagtggagaaccaggaacagaattaaagtcaccacacataacaatagggcagaagctgccatctttctggtgggcaacactggaaatctctgccagtagcattgccaattgcgtcagcttaatatcacctcgccttggattatacaacagatgcgtatttgctacgcagattgcagggcaggcagcatatggaattttgggctgtaagagtaaaactaatccaacattgtctctgtccaacagagaaatatcagggcggaagaattccactgggttcactgacaagagtgaaaatttggaatgtttgaagcaaatagcacagccatcaggtttccttcctgtccgcatcttatattcacagtgataacccagtgattccaaacttggcctgatctctgctccataatgatcttcttgaacttcttgcaaacaaagtacgtctgcatcaaaatgtttaatttctttcagaatattgggaaacctaaaactccagtgtaatactggccgccggcaatgtctataaaggtgagagttatcttccagtaaatcttgtgaaagtatattataggacatcactgaaaagtcaaacttgttctcactgtcttcacatttgggatcaacatttttgtctcctaggatcttcgttttttctttatcatggctacatatatattcccaattccgctttatcacactgcggagaggcggcctccccgccgacgctcggttcccgggacggtgctgcggagtgtgtggagcaggccagcgctggtctggaggctgggttgggggaagcaggccagggatccaaagccactggcacaagcctggccggcggcccatgaactccgcgccaagaccccagacctcgttggcccagcgtcccgccagctgcgcggcgggtttacctatcccgcttggtctctggaggctcgtcccggatgcaccatcgcccagaccctcttcctcttccttc

SEQ ID NO: 18306 - RNA, 2262 nt, Homo sapiens
  source 1..2262: mol_type = other RNA
tgaagtaccagctactcgagaggctgaggcaggagaatcgcttgagcccgggaggcaggggttgcagtgagcaaagattgcgccattgcacccccagcctgggcaacaagagtgaaactccatctcaaaaaataaaataaaataaaaataaataaataaaaatgctagggaaacaaaggtatatccccagtctctgcctctattaagcccacctcttgtctgttccagggtgaaagagtgagctttacacgttatgctggcttatatttcccaaacatttccccaacacgatgcaggcatattacatggctcaggacagtaataagatggattaagcattctgtacaacttaaaaagcattatcaaaccccttcaaaaacaaactaaacaatggctggttggatacctgtgaatgacccaaggctttctaagataaactatttagaactcaatagaggggtctcctaatgaaatcaagccttctggaaaggaaacaacttgtagtttgcaagaactcaaagatactttggatccactacagagcttgccaaaattatgaaatgaaattttttactaagcagacaaaggaagatgcattatatttaaaaatcactgtcaattttactaggatttagaatataaaacctttacatctcttttacaataaagagaatttagagctcacttgtcacgaaaatatttttcattattaaaaaaaattgttataaagttatttcttctgatatggagtttcaaagcatctaacataaccgcttcagaatctccacagtgcaaaaataaacaacatgcatacacttaagaactttacattctttgaaaaacaatacaaattggaaagaaaattagtatgtgatcaaagagagtcagagctcaagtctgaactttgccaataaaggcagatgatctgaagagttattttcgtttggaagtccattaacagtccataagtcttgttctgtaagaagtgacagtctagctagaagtttcaagccaccaaccaaagcaacttcagctcctgggtgcccagcaacatcttccttttctgcagagtagaaaatataatccacagttatggcacttcgggaatgacaggtggtcacttctggaattccagtgtcaggaaagtaatgtgaataaacagatgacaaactgaaatggtgctgtaaatttgaagacaatttttcagctgtcactaggacctctgtttgcttcagctgtgtttgtgtcagatcactgtctttcctatgggaagtccttcataattcaattttccttcctttatgaaactatatagtggagaaccaggaacagaattaaagtcaccacacataacaatagggcagaagctgccatctttctggtgggcaacactggaaatctctgccagtagcattgccaattgcgtcagcttaatatcacctcgccttggattatacaacagatgcgtatttgctacgcagattgcagggcaggcagcatatggaattttgggctgtaagagtaaaactaatccaacattgtctctgtccaacagagaaatatcagggcggaagaattccactgggttcactgacaagagtgaaaatttggaatgtttgaagcaaatagcacagccatcaggtttccttcctgtccgcatcttatattcacagtgataacccagtgattccaaacttggcctgatctctgctccataatgatcttcttgaacttcttgcaaacaaagtacgtctgcatcaaaatgtttaatttctttcagaatattgggaaacctaaaactccagtgtaatactggccgccggcaatgtctataaaggtgagagttatcttccagtaaatcttgtgaaagtatattataggacatcactgaaaagtcaaacttgttctcactgtcttcacatttgggatcaacatttttgtctcctaggatcttcgttttttctttatcatggctacatatatattcccaattccgctttatcacaccggcctcttcccaccacacagtggccgtagcccttcctcacacagcgccaggcttccatcttcgccctccgcgtgcgtccagttcccaggccccgggttccacctcaatctctataatcgatgcgacggcctaaagtatctagggaaccccatcactcttaagtaccgactccagtcctggctgcaaggcatgctgggaggtgcagtctcgccggccggcctacactccatcttgcgcagtcagagtccctgaat

SEQ ID NO: 18307 - RNA, 2837 nt, Homo sapiens
  source 1..2837: mol_type = other RNA
tgaagtaccagctactcgagaggctgaggcaggagaatcgcttgagcccgggaggcaggggttgcagtgagcaaagattgcgccattgcacccccagcctgggcaacaagagtgaaactccatctcaaaaaataaaataaaataaaaataaataaataaaaatgctagggaaacaaaggtatatccccagtctctgcctctattaagcccacctcttgtctgttccagggtgaaagagtgagctttacacgttatgctggcttatatttcccaaacatttccccaacacgatgcaggcatattacatggctcaggacagtaataagatggattaagcattctgtacaacttaaaaagcattatcaaaccccttcaaaaacaaactaaacaatggctggttggatacctgtgaatgacccaaggctttctaagataaactatttagaactcaatagaggggtctcctaatgaaatcaagccttctggaaaggaaacaacttgtagtttgcaagaactcaaagatactttggatccactacagagcttgccaaaattatgaaatgaaattttttactaagcagacaaaggaagatgcattatatttaaaaatcactgtcaattttactaggatttagaatataaaacctttacatctcttttacaataaagagaatttagagctcacttgtcacgaaaatatttttcattattaaaaaaaattgttataaagttatttcttctgatatggagtttcaaagcatctaacataaccgcttcagaatctccacagtgcaaaaataaacaacatgcatacacttaagaactttacattctttgaaaaacaatacaaattggaaagaaaattagtatgtgatcaaagagagtcagagctcaagtctgaactttgccaataaaggcagatgatctgaagagttattttcgtttggaagtccattaacagtccataagtcttgttctgtaagaagtgacagtctagctagaagtttcaagccaccaaccaaagcaacttcagctcctgggtgcccagcaacatcttccttttctgcagagtagaaaatataatccacagttatggcacttcgggaatgacaggtggtcacttctggaattccagtgtcaggaaagtaatgtgaataaacagatgacaaactgaaatggtgctgtaaatttgaagacaatttttcagctgtcactaggacctctgtttgcttcagctgtgtttgtgtcagatcactgtctttcctatgggaagtccttcataattcaattttccttcctttatgaaactatatagtggagaaccaggaacagaattaaagtcaccacacataacaatagggcagaagctgccatctttctggtgggcaacactggaaatctctgccagtagcattgccaattgcgtcagcttaatatcacctcgccttggattatacaacagatgcgtatttgctacgcagattgcagggcaggcagcatatggaattttgggctgtaagagtaaaactaatccaacattgtctctgtccaacagagaaatatcagggcggaagaattccactgggttcactgacaagagtgaaaatttggaatgtttgaagcaaatagcacagccatcaggtttccttcctgtccgcatcttatattcacagtgataacccagtgattccaaacttggcctgatctctgctccataatgatcttcttgaacttcttgcaaacaaagtacgtctgcatcaaaatgtttaatttctttcagaatattgggaaacctaaaactccagtgtaatactggccgccggcaatgtctataaaggtgagagttatcttccagtaaatcttgtgaaagtatattataggacatcactgaaaagtcaaacttgttctcactgtcttcacatttgggatcaacatttttgtctcctaggatcttcgttttttctttatcatggctacatatatattcccaattccgctttatcacaccttccatatcaggaggaacaaggtgatcacagcagagaagacagatgaatcaaagaaagtaagcaataggcctgatcaggtttttagggtgcctaattacaaagtcataattgtatcacacaaatccttcaaataccactttaaagtgataggcaagttagcaatgctgttttcttgattgaaaagtattagtgaaatatcggaagtcacaaatatggcttaacgaagagcattttccttattcacaacaccttggtgttttcttcgttttgatgaaggctcatctccctcagcgttcatgacgtaactagagagatgaatcaaagatgtctggctcaggttgtcaggtctccagttacagtactggaactgagttctagactcaaacaaacagggtggtctccaatttagtgaaaaatgcctactactgaagtatgggtaaggagctcgagagtaatgtccaggccacctcatacaactagaaatatgtctgttccagcaacacctttgcagattctcccacggtgtagtccagtctctgcccagactcctcgagtgatggggaaacatggggtatcggcctcttcccaccacacagtggccgtagcccttcctcacacagcgccaggcttccatcttcgccctccgcgtgcgtccagttcccaggccccgggttccacctcaatctctataatcgatgcgacggcctaaagtatctagggaaccccatcactcttaagtaccgactccagtcctggctgcaaggcatgctgggaggtgcagtctcgccggccggcctacactccatcttgcgcagtcagagtccctga

SEQ ID NO: 18308 - RNA, 2836 nt, Homo sapiens
  source 1..2836: mol_type = other RNA
tgaagtaccagctactcgagaggctgaggcaggagaatcgcttgagcccgggaggcaggggttgcagtgagcaaagattgcgccattgcacccccagcctgggcaacaagagtgaaactccatctcaaaaaataaaataaaataaaaataaataaataaaaatgctagggaaacaaaggtatatccccagtctctgcctctattaagcccacctcttgtctgttccagggtgaaagagtgagctttacacgttatgctggcttatatttcccaaacatttccccaacacgatgcaggcatattacatggctcaggacagtaataagatggattaagcattctgtacaacttaaaaagcattatcaaaccccttcaaaaacaaactaaacaatggctggttggatacctgtgaatgacccaaggctttctaagataaactatttagaactcaatagaggggtctcctaatgaaatcaagccttctggaaaggaaacaacttgtagtttgcaagaactcaaagatactttggatccactacagagcttgccaaaattatgaaatgaaattttttactaagcagacaaaggaagatgcattatatttaaaaatcactgtcaattttactaggatttagaatataaaacctttacatctcttttacaataaagagaatttagagctcacttgtcacgaaaatatttttcattattaaaaaaaattgttataaagttatttcttctgatatggagtttcaaagcatctaacataaccgcttcagaatctccacagtgcaaaaataaacaacatgcatacacttaagaactttacattctttgaaaaacaatacaaattggaaagaaaattagtatgtgatcaaagagagtcagagctcaagtctgaactttgccaataaaggcagatgatctgaagagttattttcgtttggaagtccattaacagtccataagtcttgttctgtaagaagtgacagtctagctagaagtttcaagccaccaaccaaagcaacttcagctcctgggtgcccagcaacatcttccttttctgcagagtagaaaatataatccacagttatggcacttcgggaatgacaggtggtcacttctggaattccagtgtcaggaaagtaatgtgaataaacagatgacaaactgaaatggtgctgtaaatttgaagacaatttttcagctgtcactaggacctctgtttgcttcagctgtgtttgtgtcagatcactgtctttcctatgggaagtccttcataattcaattttccttcctttatgaaactatatagtggagaaccaggaacagaattaaagtcaccacacataacaatagggcagaagctgccatctttctggtgggcaacactggaaatctctgccagtagcattgccaattgcgtcagcttaatatcacctcgccttggattatacaacagatgcgtatttgctacgcagattgcagggcaggcagcatatggaattttgggctgtaagagtaaaactaatccaacattgtctctgtccaacagagaaatatcagggcggaagaattccactgggttcactgacaagagtgaaaatttggaatgtttgaagcaaatagcacagccatcaggtttccttcctgtccgcatcttatattcacagtgataacccagtgattccaaacttggcctgatctctgctccataatgatcttcttgaacttcttgcaaacaaagtacgtctgcatcaaaatgtttaatttctttcagaatattgggaaacctaaaactccagtgtaatactggccgccggcaatgtctataaaggtgagagttatcttccagtaaatcttgtgaaagtatattataggacatcactgaaaagtcaaacttgttctcactgtcttcacatttgggatcaacatttttgtctcctaggatcttcgttttttctttatcatggctacatatatattcccaattccgctttatcacaccttccatatcaggaggaacaaggtgatcacagcagagaagacagatgaatcaaagaaagtaagcaataggcctgatcaggtttttagggtgcctaattacaaagtcataattgtatcacacaaatccttcaaataccactttaaagtgataggcaagttagcaatgctgttttcttgattgaaaagtattagtgaaatatcggaagtcacaaatatggcttaacgaagagcattttccttattcacaacaccttggtgttttcttcgttttgatgaaggctcatctccctcagcgttcatgacgtaactagagagatgaatcaaagatgtctggctcaggttgtcaggtctccagttacagtactggaactgagttctagactcaaacaaacagggtggtctccaatttagtgaaaaatgcctactactgaagtatgggtaaggagctcgagagtaatgtccaggccacctcatacaactagaaatatgtctgttccagcaacacctttgcagattctcccacggtgtagtccagtctctgcccagactcctcgagtgatggggaaacatggggtattgcggagaggcggcctccccgccgacgctcggttcccgggacggtgctgcggagtgtgtggagcaggccagcgctggtctggaggctgggttgggggaagcaggccagggatccaaagccactggcacaagcctggccggcggcccatgaactccgcgccaagaccccagacctcgttggcccagcgtcccgccagctgcgcggcgggtttacctatcccgcttggtctctggaggctcgtcccggatgcac

SEQ ID NO: 18309 - RNA, 2545 nt, Homo sapiens
  source 1..2545: mol_type = other RNA
tgaagtaccagctactcgagaggctgaggcaggagaatcgcttgagcccgggaggcaggggttgcagtgagcaaagattgcgccattgcacccccagcctgggcaacaagagtgaaactccatctcaaaaaataaaataaaataaaaataaataaataaaaatgctagggaaacaaaggtatatccccagtctctgcctctattaagcccacctcttgtctgttccagggtgaaagagtgagctttacacgttatgctggcttatatttcccaaacatttccccaacacgatgcaggcatattacatggctcaggacagtaataagatggattaagcattctgtacaacttaaaaagcattatcaaaccccttcaaaaacaaactaaacaatggctggttggatacctgtgaatgacccaaggctttctaagataaactatttagaactcaatagaggggtctcctaatgaaatcaagccttctggaaaggaaacaacttgtagtttgcaagaactcaaagatactttggatccactacagagcttgccaaaattatgaaatgaaattttttactaagcagacaaaggaagatgcattatatttaaaaatcactgtcaattttactaggatttagaatataaaacctttacatctcttttacaataaagagaatttagagctcacttgtcacgaaaatatttttcattattaaaaaaaattgttataaagttatttcttctgatatggagtttcaaagcatctaacataaccgcttcagaatctccacagtgcaaaaataaacaacatgcatacacttaagaactttacattctttgaaaaacaatacaaattggaaagaaaattagtatgtgatcaaagagagtcagagctcaagtctgaactttgccaataaaggcagatgatctgaagagttattttcgtttggaagtccattaacagtccataagtcttgttctgtaagaagtgacagtctagctagaagtttcaagccaccaaccaaagcaacttcagctcctgggtgcccagcaacatcttccttttctgcagagtagaaaatataatccacagttatggcacttcgggaatgacaggtggtcacttctggaattccagtgtcaggaaagtaatgtgaataaacagatgacaaactgaaatggtgctgtaaatttgaagacaatttttcagctgtcactaggacctctgtttgcttcagctgtgtttgtgtcagatcactgtctttcctatgggaagtccttcataattcaattttccttcctttatgaaactatatagtggagaaccaggaacagaattaaagtcaccacacataacaatagggcagaagctgccatctttctggtgggcaacactggaaatctctgccagtagcattgccaattgcgtcagcttaatatcacctcgccttggattatacaacagatgcgtatttgctacgcagattgcagggcaggcagcatatggaattttgggctgtaagagtaaaactaatccaacattgtctctgtccaacagagaaatatcagggcggaagaattccactgggttcactgacaagagtgaaaatttggaatgtttgaagcaaatagcacagccatcaggtttccttcctgtccgcatcttatattcacagtgataacccagtgattccaaacttggcctgatctctgctccataatgatcttcttgaacttcttgcaaacaaagtacgtctgcatcaaaatgtttaatttctttcagaatattgggaaacctaaaactccagtgtaatactggccgccggcaatgtctataaaggtgagagttatcttccagtaaatcttgtgaaagtatattataggacatcactgaaaagtcaaacttgttctcactgtcttcacatttgggatcaacatttttgtctcctaggatcttcgttttttctttatcatggctacatatatattcccaattccgctttatcacaccttggtgttttcttcgttttgatgaaggctcatctccctcagcgttcatgacgtaactagagagatgaatcaaagatgtctggctcaggttgtcaggtctccagttacagtactggaactgagttctagactcaaacaaacagggtggtctccaatttagtgaaaaatgcctactactgaagtatgggtaaggagctcgagagtaatgtccaggccacctcatacaactagaaatatgtctgttccagcaacacctttgcagattctcccacggtgtagtccagtctctgcccagactcctcgagtgatggggaaacatggggtatacagcgccaggcttccatcttcgccctccgcgtgcgtccagttcccaggccccgggttccacctcaatctctataatcgatgcgacggcctaaagtatctagggaaccccatcactcttaagtaccgactccagtcctggctgcaaggcatgctgggaggtgcagtctcgccggccggcctacactccatcttgcgcagtcagagtccctga

SEQ ID NO: 18310 - RNA, 2516 nt, Homo sapiens
  source 1..2516: mol_type = other RNA
tgaagtaccagctactcgagaggctgaggcaggagaatcgcttgagcccgggaggcaggggttgcagtgagcaaagattgcgccattgcacccccagcctgggcaacaagagtgaaactccatctcaaaaaataaaataaaataaaaataaataaataaaaatgctagggaaacaaaggtatatccccagtctctgcctctattaagcccacctcttgtctgttccagggtgaaagagtgagctttacacgttatgctggcttatatttcccaaacatttccccaacacgatgcaggcatattacatggctcaggacagtaataagatggattaagcattctgtacaacttaaaaagcattatcaaaccccttcaaaaacaaactaaacaatggctggttggatacctgtgaatgacccaaggctttctaagataaactatttagaactcaatagaggggtctcctaatgaaatcaagccttctggaaaggaaacaacttgtagtttgcaagaactcaaagatactttggatccactacagagcttgccaaaattatgaaatgaaattttttactaagcagacaaaggaagatgcattatatttaaaaatcactgtcaattttactaggatttagaatataaaacctttacatctcttttacaataaagagaatttagagctcacttgtcacgaaaatatttttcattattaaaaaaaattgttataaagttatttcttctgatatggagtttcaaagcatctaacataaccgcttcagaatctccacagtgcaaaaataaacaacatgcatacacttaagaactttacattctttgaaaaacaatacaaattggaaagaaaattagtatgtgatcaaagagagtcagagctcaagtctgaactttgccaataaaggcagatgatctgaagagttattttcgtttggaagtccattaacagtccataagtcttgttctgtaagaagtgacagtctagctagaagtttcaagccaccaaccaaagcaacttcagctcctgggtgcccagcaacatcttccttttctgcagagtagaaaatataatccacagttatggcacttcgggaatgacaggtggtcacttctggaattccagtgtcaggaaagtaatgtgaataaacagatgacaaactgaaatggtgctgtaaatttgaagacaatttttcagctgtcactaggacctctgtttgcttcagctgtgtttgtgtcagatcactgtctttcctatgggaagtccttcataattcaattttccttcctttatgaaactatatagtggagaaccaggaacagaattaaagtcaccacacataacaatagggcagaagctgccatctttctggtgggcaacactggaaatctctgccagtagcattgccaattgcgtcagcttaatatcacctcgccttggattatacaacagatgcgtatttgctacgcagattgcagggcaggcagcatatggaattttgggctgtaagagtaaaactaatccaacattgtctctgtccaacagagaaatatcagggcggaagaattccactgggttcactgacaagagtgaaaatttggaatgtttgaagcaaatagcacagccatcaggtttccttcctgtccgcatcttatattcacagtgataacccagtgattccaaacttggcctgatctctgctccataatgatcttcttgaacttcttgcaaacaaagtacgtctgcatcaaaatgtttaatttctttcagaatattgggaaacctaaaactccagtgtaatactggccgccggcaatgtctataaaggtgagagttatcttccagtaaatcttgtgaaagtatattataggacatcactgaaaagtcaaacttgttctcactgtcttcacatttgggatcaacatttttgtctcctaggatcttcgttttttctttatcatggctacatatatattcccaattccgctttatcacaccttggtgttttcttcgttttgatgaaggctcatctccctcagcgttcatgacgtaactagagagatgaatcaaagatgtctggctcaggttgtcaggtctccagttacagtactggaactgagttctagactcaaacaaacagggtggtctccaatttagtgaaaaatgcctactactgaagtatgggtaaggagctcgagagtaatgtccaggccacctcatacaactagaaatatgtctgttccagcaacacctttgcagattctcccacggtgtagtccagtctctgcccagactcctcgagtgatggggaaacatggggtatcggcctcttcccaccacacagtggccgtagcccttcctcacacagcgccaggcttccatcttcgccctccgcgtgcgtccagttcccaggccccgggttccacctcaatctctataatcgatgcgacggcctaaagtatctagggaaccccatcactcttaagtaccgactccagtcctggct

SEQ ID NO: 18311 - RNA, 2406 nt, Homo sapiens
  source 1..2406: mol_type = other RNA
tgaagtaccagctactcgagaggctgaggcaggagaatcgcttgagcccgggaggcaggggttgcagtgagcaaagattgcgccattgcacccccagcctgggcaacaagagtgaaactccatctcaaaaaataaaataaaataaaaataaataaataaaaatgctagggaaacaaaggtatatccccagtctctgcctctattaagcccacctcttgtctgttccagggtgaaagagtgagctttacacgttatgctggcttatatttcccaaacatttccccaacacgatgcaggcatattacatggctcaggacagtaataagatggattaagcattctgtacaacttaaaaagcattatcaaaccccttcaaaaacaaactaaacaatggctggttggatacctgtgaatgacccaaggctttctaagataaactatttagaactcaatagaggggtctcctaatgaaatcaagccttctggaaaggaaacaacttgtagtttgcaagaactcaaagatactttggatccactacagagcttgccaaaattatgaaatgaaattttttactaagcagacaaaggaagatgcattatatttaaaaatcactgtcaattttactaggatttagaatataaaacctttacatctcttttacaataaagagaatttagagctcacttgtcacgaaaatatttttcattattaaaaaaaattgttataaagttatttcttctgatatggagtttcaaagcatctaacataaccgcttcagaatctccacagtgcaaaaataaacaacatgcatacacttaagaactttacattctttgaaaaacaatacaaattggaaagaaaattagtatgtgatcaaagagagtcagagctcaagtctgaactttgccaataaaggcagatgatctgaagagttattttcgtttggaagtccattaacagtccataagtcttgttctgtaagaagtgacagtctagctagaagtttcaagccaccaaccaaagcaacttcagctcctgggtgcccagcaacatcttccttttctgcagagtagaaaatataatccacagttatggcacttcgggaatgacaggtggtcacttctggaattccagtgtcaggaaagtaatgtgaataaacagatgacaaactgaaatggtgctgtaaatttgaagacaatttttcagctgtcactaggacctctgtttgcttcagctgtgtttgtgtcagatcactgtctttcctatgggaagtccttcataattcaattttccttcctttatgaaactatatagtggagaaccaggaacagaattaaagtcaccacacataacaatagggcagaagctgccatctttctggtgggcaacactggaaatctctgccagtagcattgccaattgcgtcagcttaatatcacctcgccttggattatacaacagatgcgtatttgctacgcagattgcagggcaggcagcatatggaattttgggctgtaagagtaaaactaatccaacattgtctctgtccaacagagaaatatcagggcggaagaattccactgggttcactgacaagagtgaaaatttggaatgtttgaagcaaatagcacagccatcaggtttccttcctgtccgcatcttatattcacagtgataacccagtgattccaaacttggcctgatctctgctccataatgatcttcttgaacttcttgcaaacaaagtacgtctgcatcaaaatgtttaatttctttcagaatattgggaaacctaaaactccagtgtaatactggccgccggcaatgtctataaaggtgagagttatcttccagtaaatcttgtgaaagtatattataggacatcactgaaaagtcaaacttgttctcactgtcttcacatttgggatcaacatttttgtctcctaggatcttcgttttttctttatcatggctacatatatattcccaattccgctttatcacaccttggtgttttcttcgttttgatgaaggctcatctccctcagcgttcatgacgtaactagagagatgaatcaaagatgtctggctcaggttgtcaggtctccagttacagtactggaactgagttctagactcaaacaaacagggtggtctccaatttagtgaaaaatgcctactactgaagtatgggtaaggagctcgagagtaatgtccaggccacctcatacaactagaaatatgtctgttccagcaacacctttgcagattctcccacggtgtagtccagtctctgcccagactcctcgagtgatggggaaacatggggtatctatcccgcttggtctctggaggctcgtcccggatgcaccatcgcccagaccctcttcctcttccttccaccc

SEQ ID NO: 18312 - RNA, 2617 nt, Homo sapiens
  source 1..2617: mol_type = other RNA
tgaagtaccagctactcgagaggctgaggcaggagaatcgcttgagcccgggaggcaggggttgcagtgagcaaagattgcgccattgcacccccagcctgggcaacaagagtgaaactccatctcaaaaaataaaataaaataaaaataaataaataaaaatgctagggaaacaaaggtatatccccagtctctgcctctattaagcccacctcttgtctgttccagggtgaaagagtgagctttacacgttatgctggcttatatttcccaaacatttccccaacacgatgcaggcatattacatggctcaggacagtaataagatggattaagcattctgtacaacttaaaaagcattatcaaaccccttcaaaaacaaactaaacaatggctggttggatacctgtgaatgacccaaggctttctaagataaactatttagaactcaatagaggggtctcctaatgaaatcaagccttctggaaaggaaacaacttgtagtttgcaagaactcaaagatactttggatccactacagagcttgccaaaattatgaaatgaaattttttactaagcagacaaaggaagatgcattatatttaaaaatcactgtcaattttactaggatttagaatataaaacctttacatctcttttacaataaagagaatttagagctcacttgtcacgaaaatatttttcattattaaaaaaaattgttataaagttatttcttctgatatggagtttcaaagcatctaacataaccgcttcagaatctccacagtgcaaaaataaacaacatgcatacacttaagaactttacattctttgaaaaacaatacaaattggaaagaaaattagtatgtgatcaaagagagtcagagctcaagtctgaactttgccaataaaggcagatgatctgaagagttattttcgtttggaagtccattaacagtccataagtcttgttctgtaagaagtgacagtctagctagaagtttcaagccaccaaccaaagcaacttcagctcctgggtgcccagcaacatcttccttttctgcagagtagaaaatataatccacagttatggcacttcgggaatgacaggtggtcacttctggaattccagtgtcaggaaagtaatgtgaataaacagatgacaaactgaaatggtgctgtaaatttgaagacaatttttcagctgtcactaggacctctgtttgcttcagctgtgtttgtgtcagatcactgtctttcctatgggaagtccttcataattcaattttccttcctttatgaaactatatagtggagaaccaggaacagaattaaagtcaccacacataacaatagggcagaagctgccatctttctggtgggcaacactggaaatctctgccagtagcattgccaattgcgtcagcttaatatcacctcgccttggattatacaacagatgcgtatttgctacgcagattgcagggcaggcagcatatggaattttgggctgtaagagtaaaactaatccaacattgtctctgtccaacagagaaatatcagggcggaagaattccactgggttcactgacaagagtgaaaatttggaatgtttgaagcaaatagcacagccatcaggtttccttcctgtccgcatcttatattcacagtgataacccagtgattccaaacttggcctgatctctgctccataatgatcttcttgaacttcttgcaaacaaagtacgtctgcatcaaaatgtttaatttctttcagaatattgggaaacctaaaactccagtgtaatactggccgccggcaatgtctataaaggtgagagttatcttccagtaaatcttgtgaaagtatattataggacatcactgaaaagtcaaacttgttctcactgtcttcacatttgggatcaacatttttgtctcctaggatcttcgttttttctttatcatggctacatatatattcccaattccgctttatcacaccttggtgttttcttcgttttgatgaaggctcatctccctcagcgttcatgacgtaactagagagatgaatcaaagatgtctggctcaggttgtcaggtctccagttacagtactggaactgagttctagactcaaacaaacagggtggtctccaatttagtgaaaaatgcctactactgaagtatgggtaaggagctcgagagtaatgtccaggccacctcatacaactagaaatatgtctgttccagcaacacctttgcagattctcccacggtgtagtccagtctctgcccagactcctcgagtgatggggaaacatggggtattgcggagaggcggcctccccgccgacgctcggttcccgggacggtgctgcggagtgtgtggagcaggccagcgctggtctggaggctgggttgggggaagcaggccagggatccaaagccactggcacaagcctggccggcggcccatgaactccgcgccaagaccccagacctcgttggcccagcgtcccgccagctgcgcggcgggtttacctatcccgcttggtctctggaggctcgtcccggatgcaccatcgcccagaccctcttcctcttccttccac

SEQ ID NO: 18313 - RNA, 2284 nt, Homo sapiens
  source 1..2284: mol_type = other RNA
tgaagtaccagctactcgagaggctgaggcaggagaatcgcttgagcccgggaggcaggggttgcagtgagcaaagattgcgccattgcacccccagcctgggcaacaagagtgaaactccatctcaaaaaataaaataaaataaaaataaataaataaaaatgctagggaaacaaaggtatatccccagtctctgcctctattaagcccacctcttgtctgttccagggtgaaagagtgagctttacacgttatgctggcttatatttcccaaacatttccccaacacgatgcaggcatattacatggctcaggacagtaataagatggattaagcattctgtacaacttaaaaagcattatcaaaccccttcaaaaacaaactaaacaatggctggttggatacctgtgaatgacccaaggctttctaagataaactatttagaactcaatagaggggtctcctaatgaaatcaagccttctggaaaggaaacaacttgtagtttgcaagaactcaaagatactttggatccactacagagcttgccaaaattatgaaatgaaattttttactaagcagacaaaggaagatgcattatatttaaaaatcactgtcaattttactaggatttagaatataaaacctttacatctcttttacaataaagagaatttagagctcacttgtcacgaaaatatttttcattattaaaaaaaattgttataaagttatttcttctgatatggagtttcaaagcatctaacataaccgcttcagaatctccacagtgcaaaaataaacaacatgcatacacttaagaactttacattctttgaaaaacaatacaaattggaaagaaaattagtatgtgatcaaagagagtcagagctcaagtctgaactttgccaataaaggcagatgatctgaagagttattttcgtttggaagtccattaacagtccataagtcttgttctgtaagaagtgacagtctagctagaagtttcaagccaccaaccaaagcaacttcagctcctgggtgcccagcaacatcttccttttctgcagagtagaaaatataatccacagttatggcacttcgggaatgacaggtggtcacttctggaattccagtgtcaggaaagtaatgtgaataaacagatgacaaactgaaatggtgctgtaaatttgaagacaatttttcagctgtcactaggacctctgtttgcttcagctgtgtttgtgtcagatcactgtctttcctatgggaagtccttcataattcaattttccttcctttatgaaactatatagtggagaaccaggaacagaattaaagtcaccacacataacaatagggcagaagctgccatctttctggtgggcaacactggaaatctctgccagtagcattgccaattgcgtcagcttaatatcacctcgccttggattatacaacagatgcgtatttgctacgcagattgcagggcaggcagcatatggaattttgggctgtaagagtaaaactaatccaacattgtctctgtccaacagagaaatatcagggcggaagaattccactgggttcactgacaagagtgaaaatttggaatgtttgaagcaaatagcacagccatcaggtttccttcctgtccgcatcttatattcacagtgataacccagtgattccaaacttggcctgatctctgctccataatgatcttcttgaacttcttgcaaacaaagtacgtctgcatcaaaatgtttaatttctttcagaatattgggaaacctaaaactccagtgtaatactggccgccggcaatgtctataaaggtgagagttatcttccagtaaatcttgtgaaagtatattataggacatcactgaaaagtcaaacttgttctcactgtcttcacatttgggatcaacatttttgtctcctaggatcttcgttttttctttatcatggctacatatatattcccaattccgctttatcacactgcggagaggcggcctccccgccgacgctcggttcccgggacggtgctgcggagtgtgtggagcaggccagcgctggtctggaggctgggttgggggaagcaggccagggatccaaagccactggcacaagcctggccggcggcccatgaactccgcgccaagaccccagacctcgttggcccagcgtcccgccagctgcgcggcgggtttacctatcccgcttggtctctggaggctcgtcccggatgcaccatcgcccagaccctcttcctcttc

SEQ ID NO: 18314 - RNA, 263 nt, Homo sapiens
  source 1..263: mol_type = other RNA
tgaagtaccagctactcgagaggctgaggcaggagaatcggttgaacccgggaagcggaggttgcagtgagccgagatcacgccattgcactccagcctgggtgtcgcagtgacagtgattcatgggaatcgatgattgatgatttcgatagttcggtaatcgctaatgggcaggcgccgggcgaccagtacttgatgaccgcgatgttgaccggcgctgtacaagtgactgccgccagcggcttctccgaggccatggtccc

SEQ ID NO: 18315 - RNA, 1786 nt, Homo sapiens
  source 1..1786: mol_type = other RNA
tgaagtaccagctactcgagaggctgaggcaggagaatggcgtgaacctgggaggcgcagcttgcagtaagccgagatcgcgccactgcactccagcctgggtgacagaacgagactccatctcaaaaaaaaaaaagaagggggcacagggagtacaggggaaggggaggaggctgtagctgttccatcattggtgacctgtactgggtagatggtgactagcagtgcgtgatgctacagcaagccatgccctccccaccccaccctgcgctgggacccttgggcctgccataagtcatagtccacactcactggaggggtccactctattgttgtgtcctgaccacatccttgctaagacccaggctcttctttctcctagtagctccgtgatgaacacaaatgcccttctcctgtcggaccctccagacactccagtccagtctaccttgggattgcggtcattactctcctcttgactttccttgtgcttcttgttctgtcctggtctctgtcagtcctttccctgtctgacgcgagtcccagctccttataccactcctgggaattctccagttcctgactcactgtctgcagcctgcaggctctgacagcaccgcaggtgtcagaaggcgcctcttatgttcaagggtcctgggcttccagcatgggagtagacggcaagttaccagtggccccaaatgttagatactgtggcttgattacagagaaataggagacagctccatgagatccaacagatggtctgattagggaagaaggaagccagtgcagaacacttacaaaataaccatgcttgatagtgagctgttttggacagggacggtttggcaggcccttctgaaatcttcacagccggcgtcaggcctggcactcagcagcacgcaacaaataattgttaaatgaataaataaaacataagggctggacacagtggctcacacctgtaatcccagcactttgggaggctgaggcgggtggattgcttgaggccaggtgtttgagaccagcctagccaacatgacaaaaccccgtctctgctaaaaatattatacaaaaattagccaggcgcggcgaagagtgcctgtaatctcagctacttagaaggctgaggcaggagaattacttgaacccaggaggcagaggttacagttagccaagatcgtgccactacactccagcctgggtgactctgtggtccgagctactcgagaggcagacgtgggaggatgtcttgagcccaggaggttaaggctgcagtgagctgtgattgtaccactgcactccagcctggacaacagaacaagatcccgattcttggtggtattcagagaggtttggtctgactgagctgcagcagctgtccgactcccaggggaaaaagcgaaaggctgagagaatcccagacactggcctgacacgttggaactgccgaaattccatgaaggatccagataatggccatcacatcatcatttaaggcaggacgtaaggactaaccatgtctcttctccagctctacatatttcatcctgagcagcaagggaggctgagaaagtgggcgctggagccttggcagcctctgttaagagggtcatccagggcttccttgccgcctcggtgcacagctcaatcatgcttccttcttgttcattttgacaaagcaggtgagtgatgagcaggaaaaaattatgaggaggtgttggagcaactcgctaatcagcactgctacaagatcgccagcatttacaggaccgcattcact

SEQ ID NO: 18316 - RNA, 3766 nt, Homo sapiens
  source 1..3766: mol_type = other RNA
tgaagtaccagctactcgagaggctgaggcaggagaattgcttgaaccaaggaggcagaggttgcagtgagccaagaccacgccaacgcactccagcctgggcaacaagagtgaaactccatctcaaaaaagaaaaaaaaaaaaaaaaggccgggcgtggtggctcacatctgtaatcctagcacttggggaggccgaggcaggcagattacctgagttcaggagttttagaacagcctgggcaacacggtgaaaccccgtctctactaaaatgcaaaaaattagctgggcgtggcagtgtgtgcctgcagtcccagctactcgggaggctgaggcaggataattgcttgcacccaggaggcagaggttgcagtgagccgagatcgtgccaccgcactccaccctgcgcgacagagcaaaactccgtctcaaaataaaaaaaaataaaaaataaaaaaatctgtgttaaataactaaagttgaaaattgaatgtcagttttattatggtggattttctcccgtgtcttcacgactcacagcgctgagtgtgctaaccaatggtgggcttaattggggtactaggctcaggaaatagctgccattcttgctaccaagtggcctcacataattatcttaaggcatctcttgagctgaaacaggtggggctggtaattggcagcctcaagtaaaataggaggagagagaggctcagagtgggttgcagaggaactggtgaataaattcttgagccttcttcttctctgtcatatcaagcttttggtgaccagctgggtttcgaagcaataagctgccaaatatgctagctagaatattctcatccaaatgattttttgctgaatttttcagcagttctcgcaaaaacgccatcaagtagtggaagacatttttgtggaatatggggagagtagaaatgacctgtttgcttgctgtgtagttgccagaacactccaagcagttatggtaggtgctgtaacagatgacaggctctggaaggctctccaggaaaagcagcagggcttcggctacagaatgattgctggcagagaggttatcaatcattccagtatccaagcagtccctgatatgttcaaattctgacctcaggcctggttgctgaaacagatcttcctgctggacagcatttcggtacaggtaatcaaccatcatccagagctctttggggatttccatggggctatccaactggctcccatcatctccagtccatactggcatcagagtcagctcactaatggtttcaagtggtaggtccaagattggctctctcatgtaacacagtgtatgaatgggagacccaaaacagctgggcaggtagttcccagacacagacaaaaagtaatcctttcccctgtccaagtgcagaaccagaatgtcctcaattttgtcttcacccgagttgagctttgtagctgtcatcttatttacgaagagctccaagtcaatctcaacatcagaatctggcaggaggaagcctctgctggggttggcattcagccactgcttacagtaagactcttcatcaggcttgttgatgaattcaaaatgacagggtacttgtccattatgaattgtaaaggattctactttcaattgcatgtacttcacattctgaaaacagaactctcgcttggacagggacacagaaggaatgttggcattttccatcttatccagggagcgaacaatttcctccagtgtcttccggtaaagctcgtcatttacgaccctcaccccgatgtcaaacactgagctgacaggcttgtggtcactggtcttcagggccatgtggctctggtaactcagctgagtgatgttcttccctttccagagaatccgatcacaccaggcaggagcacggcacttctcactgaaatgcaaagtccacactggaagtactcacagaaacagcagtgcccgctgcctggcgagtgccctggctcaggtggggagtgatgaatcagggccttcatgtccatgtggctaagtcatctgaggcagcaagagcaattcgggcccaccaagggataacatgtatcctggtatcccagtcgtcagagcccgtatcatacttgtaagtaggctggaatgtgagctcaccctctgtgaagccttcaaagacagtctttgcggccacctgaattttcagctgatcatatgcatacagcatttgaaagtccttctcttcgatgagctttttcactttttccacatccagctcttctatcctgtagttgaggtcccccagccacaagatcacactcacaaactaggatgctgcaggttcaccagaatggaagagctcggctgcaagacactccctgctaggctcctcatggttgctgatggtgagagggggaaggcttgggtcaggctgacaaaactgcattcgagaacaaatgtccttatagtcctggttcctcctctcatactcttcaatgtgggctgccaagtgagaattcacaacgcagatgctggtgttgtggaactggaacctgatcgccacgcctcccttgttgcccatcctccccatgattcctgtccccacagtctcggcttccacttctgagatataagctgcatgctcctgtttgacatataacagcagcataatcccaaccagtcggataagcttcacctttgcatatttggcatctggatgaagaccctctgacacagctttgaaccactcttcctcctttggggtatcgtgaaagaaaaaagcttccttactcagatcaagctcctggaaccctacacaatagacatctggggcctggataccattgctcagccacagccggaggcattctttgggggactgcccatttacattgtatgttcccgcaaaaaacctgaagttctggatataggtgtaatcctcttctttctgtagtagatgtgatttcacaattgtatctcgcagtccaaacttctgcatggataaaatatgagccttgtccgacactgtgatagtggaggagcgaaccatgtcagtaatttcggacttggatttattctgtcttggttgcaagctttctggtttatcttgacccctggagctttggtccataggcactcccttcccatttggtctcaaaccatcaaagttagaaccaccctggccaggtaactagggccgagttacaaccgcgcggcgttggcatctccagctccagctctgcgcacctataccgagacagccacaggaattcaggatcccgggtcgcagaatcgaagcctggacaggccctggcaacttcgtggaggaacatcctggtttgtgaaccaaagggcagttggaatacgaggctaagctctgctgtgtccagctggacggtcacatctgagccaaggatgtagagttcaccatctggggacacttcttccagcgtaaaatcccgcgagactggcactatctggtccagagagacatcgtccccggtaatggccatcctccggtgcgtatagaggaagagagcgtgttcctggccgccgtgctccaggcggtagcgcacgagtcccaggaggcggctctgccggctgtccccctcacacagcacaccttgcaccgcgatgacgcagtattccccctcagccagcgtctcctggattgccacagactggtccatgctggcccctgctgagcgcacacaccctcctgagctgtcaccacagggcgcacgggactccgctgccccaggttccgggacagtgactacattt

SEQ ID NO: 18317 - RNA, 3207 nt, Homo sapiens
  source 1..3207: mol_type = other RNA
tgaagtaccagctactcgagaggctgaggcaggagaattgcttgaaccaaggaggcagaggttgcagtgagccaagaccacgccaacgcactccagcctgggcaacaagagtgaaactccatctcaaaaaagaaaaaaaaaaaaaaaaggccgggcgtggtggctcacatctgtaatcctagcacttggggaggccgaggcaggcagattacctgagttcaggagttttagaacagcctgggcaacacggtgaaaccccgtctctactaaaatgcaaaaaattagctgggcgtggcagtgtgtgcctgcagtcccagctactcgggaggctgaggcaggataattgcttgcacccaggaggcagaggttgcagtgagccgagatcgtgccaccgcactccaccctgcgcgacagagcaaaactccgtctcaaaataaaaaaaaataaaaaataaaaaaatctgtgttaaataactaaagttgaaaattgaatgtcagttttattatggtggattttctcccgtgtcttcacgactcacagcgctgagtgtgctaaccaatggtgggcttaattggggtactaggctcaggaaatagctgccattcttgctaccaagtggcctcacataattatcttaaggcatctcttgagctgaaacaggtggggctggtaattggcagcctcaagtaaaataggaggagagagaggctcagagtgggttgcagaggaactggtgaataaattcttgagccttcttcttctctgtcatatcaagcttttggtgaccagctgggtttcgaagcaataagctgccaaatatgctagctagaatattctcatccaaatgattttttgctgaatttttcagcagttctcgcaaaaacgccatcaagtagtggaagacatttttgtggaatatggggagagtagaaatgacctgtttgcttgctgtgtagttgccagaacactccaagcagttatggtaggtgctgtaacagatgacaggctctggaaggctctccaggaaaagcagcagggcttcggctacagaatgattgctggcagagaggttatcaatcattccagtatccaagcagtccctgatatgttcaaattctgacctcaggcctggttgctgaaacagatcttcctgctggacagcatttcggtacaggtaatcaaccatcatccagagctctttggggatttccatggggctatccaactggctcccatcatctccagtccatactggcatcagagtcagctcactaatggtttcaagtggtaggtccaagattggctctctcatgtaacacagtgtatgaatgggagacccaaaacagctgggcaggtagttcccagacacagacaaaaagtaatcctttcccctgtccaagtgcagaaccagaatgtcctcaattttgtcttcacccgagttgagctttgtagctgtcatcttatttacgaagagctccaagtcaatctcaacatcagaatctggcaggaggaagcctctgctggggttggcattcagccactgcttacagtaagactcttcatcaggcttgttgatgaattcaaaatgacagggtacttgtccattatgaattgtaaaggattctactttcaattgcatgtacttcacattctgaaaacagaactctcgcttggacagggacacagaaggaatgttggcattttccatcttatccagggagcgaacaatttcctccagtgtcttccggtaaagctcgtcatttacgaccctcaccccgatgtcaaacactgagctgacaggcttgtggtcactggtcttcagggccatgtggctctggtaactcagctgagtgatgttcttccctttccagagaatccgatcacaccaggcaggagcacggcacttctcactgaaatgcaaagtccacactggaagtactcacagaaacagcagtgcccgctgcctggcgagtgccctggctcaggtggggagtgatgaatcagggccttcatgtccatgtggctaagtcatctgaggcagcaagagcaattcgggcccaccaagggataacatgtatcctggtatcccagtcgtcagagcccgtatcatacttgtaagtaggctggaatgtgagctcaccctctgtgaagccttcaaagacagtctttgcggccacctgaattttcagctgatcatatgcatacagcatttgaaagtccttctcttcgatgagctttttcactttttccacatccagctcttctatcctgtagttgaggtcccccagccacaagatcacatcatggttgctgatggtgagagggggaaggcttgggtcaggctgacaaaactgcattcgagaacaaatgtccttatagtcctggttcctcctctcatactcttcaatgtgggctgccaagtgagaattcacaacgcagatgctggtgttgtggaactggaacctgatcgccacgcctcccttgttgcccatcctccccatgattcctgtccccacagtctcggcttccacttctgagatataagctgcatgctcctgtttgacatataacagcagcataatcccaaccagtcggataagcttcacctttgcatatttggcatctggatgaagaccctctgacacagctttgaaccactcttcctcctttggggtatcgtgaaagaaaaaagcttccttactcagatcaagctcctggaaccctacacaatagacatctggggcctggataccattgctcagccacagccggaggcattctttgggggactgcccatttacattgtatgttcccgcaaaaaacctgaagttctggatataggtgtaatcctcttctttctgtagtagatgtgatttcacaattgtatctcgcagtccaaacttctgcatggataaaatatgagccttgtccgacactgtgatagtggaggagcgaaccatgtcagtaatttcggacttggatttattctgtcttggttgcaagctttctggtttatcttgacccctggagctttggtccataggcactcccttcccatttggtctcaaaccatcaaagttagaaccacctgcagtgttgcgctcccgagagccggcggcggcagacatttccctgcctgcttcctcaagctcctcatcccgccgcccgtcccgcgcgctccgcccccagacgaacccgcccccgtgt

SEQ ID NO: 18318 - RNA, 3820 nt, Homo sapiens
  source 1..3820: mol_type = other RNA
tgaagtaccagctactcgagaggctgaggcaggagaattgcttgaaccaaggaggcagaggttgcagtgagccaagaccacgccaacgcactccagcctgggcaacaagagtgaaactccatctcaaaaaagaaaaaaaaaaaaaaaaggccgggcgtggtggctcacatctgtaatcctagcacttggggaggccgaggcaggcagattacctgagttcaggagttttagaacagcctgggcaacacggtgaaaccccgtctctactaaaatgcaaaaaattagctgggcgtggcagtgtgtgcctgcagtcccagctactcgggaggctgaggcaggataattgcttgcacccaggaggcagaggttgcagtgagccgagatcgtgccaccgcactccaccctgcgcgacagagcaaaactccgtctcaaaataaaaaaaaataaaaaataaaaaaatctgtgttaaataactaaagttgaaaattgaatgtcagttttattatggtggattttctcccgtgtcttcacgactcacagcgctgagtgtgctaaccaatggtgggcttaattggggtactaggctcaggaaatagctgccattcttgctaccaagtggcctcacataattatcttaaggcatctcttgagctgaaacaggtggggctggtaattggcagcctcaagtaaaataggaggagagagaggctcagagtgggttgcagaggaactggtgaataaattcttgagccttcttcttctctgtcatatcaagcttttggtgaccagctgggtttcgaagcaataagctgccaaatatgctagctagaatattctcatccaaatgattttttgctgaatttttcagcagttctcgcaaaaacgccatcaagtagtggaagacatttttgtggaatatggggagagtagaaatgacctgtttgcttgctgtgtagttgccagaacactccaagcagttatggtaggtgctgtaacagatgacaggctctggaaggctctccaggaaaagcagcagggcttcggctacagaatgattgctggcagagaggttatcaatcattccagtatccaagcagtccctgatatgttcaaattctgacctcaggcctggttgctgaaacagatcttcctgctggacagcatttcggtacaggtaatcaaccatcatccagagctctttggggatttccatggggctatccaactggctcccatcatctccagtccatactggcatcagagtcagctcactaatggtttcaagtggtaggtccaagattggctctctcatgtaacacagtgtatgaatgggagacccaaaacagctgggcaggtagttcccagacacagacaaaaagtaatcctttcccctgtccaagtgcagaaccagaatgtcctcaattttgtcttcacccgagttgagctttgtagctgtcatcttatttacgaagagctccaagtcaatctcaacatcagaatctggcaggaggaagcctctgctggggttggcattcagccactgcttacagtaagactcttcatcaggcttgttgatgaattcaaaatgacagggtacttgtccattatgaattgtaaaggattctactttcaattgcatgtacttcacattctgaaaacagaactctcgcttggacagggacacagaaggaatgttggcattttccatcttatccagggagcgaacaatttcctccagtgtcttccggtaaagctcgtcatttacgaccctcaccccgatgtcaaacactgagctgacaggcttgtggtcactggtcttcagggccatgtggctctggtaactcagctgagtgatgttcttccctttccagagaatccgatcacaccaggcaggagcacggcacttctcactgaaatgcaaagtccacactggaagtactcacagaaacagcagtgcccgctgcctggcgagtgccctggctcaggtggggagtgatgaatcagggccttcatgtccatgtggctaagtcatctgaggcagcaagagcaattcgggcccaccaagggataacatgtatcctggtatcccagtcgtcagagcccgtatcatacttgtaagtaggctggaatgtgagctcaccctctgtgaagccttcaaagacagtctttgcggccacctgaattttcagctgatcatatgcatacagcatttgaaagtccttctcttcgatgagctttttcactttttccacatccagctcttctatcctgtagttgaggtcccccagccacaagatcacatcatggttgctgatggtgagagggggaaggcttgggtcaggctgacaaaactgcattcgagaacaaatgtccttatagtcctggttcctcctctcatactcttcaatgtgggctgccaagtgagaattcacaacgcagatgctggtgttgtggaactggaacctgatcgccacgcctcccttgttgcccatcctccccatgattcctgtccccacagtctcggcttccacttctgagatataagctgcatgctcctgtttgacatataacagcagcataatcccaaccagtcggataagcttcacctttgcatatttggcatctggatgaagaccctctgacacagctttgaaccactcttcctcctttggggtatcgtgaaagaaaaaagcttccttactcagatcaagctcctggaaccctacacaatagacatctggggcctggataccattgctcagccacagccggaggcattctttgggggactgcccatttacattgtatgttcccgcaaaaaacctgaagttctggatataggtgtaatcctcttctttctgtagtagatgtgatttcacaattgtatctcgcagtccaaacttctgcatggataaaatatgagccttgtccgacacttggttgcaagctttctggtttatcttgacccctggagctttggtccataggcactcccttcccatttggtctcaaaccatcaaagttagaaccaccctggccaggtaactagggccgagttacaaccgcgcggcgttggcatctccagctccagctctgcgcacctataccgagacagccacaggaattcaggatcccgggtcgcagaatcgaagcctggacaggccctggcaacttcgtggaggaacatcctggtttgtgaaccaaagggcagttggaatacgaggctaagctctgctgtgtccagctggacggtcacatctgagccttgtccataaaatggagatgcaaacagtgataacctcatagagctgtgagaaaagcctgatttaggcccggtgcggtggctcatgcctgtaatcccagcactttgggaggccgaggtggggtggatcacaaggtcaggagatcgagaccatcctggccaacacggtgaaaccccgtctctacaaggatgtagagttcaccatctggggacacttcttccagcgtaaaatcccgcgagactggcactatctggtccagagagacatcgtccccggtaatggccatcctccggtgcgtatagaggaagagagcgtgttcctggccgccgtgctccaggcggtagcgcacgagtcccaggaggcggctctgccggctgtccccctcacacagcacaccttgcaccgcgatgacgcagtattccccctcagccagcgtctcctggattgccacagactggtccatgctggcccctgctgagcgcacacaccctcctgagctgtcaccacagggcgcacgggactccgctgccccaggttccgggacagtgactacattt

SEQ ID NO: 18319 - RNA, 3971 nt, Homo sapiens
  source 1..3971: mol_type = other RNA
tgaagtaccagctactcgagaggctgaggcaggagaattgcttgaaccaaggaggcagaggttgcagtgagccaagaccacgccaacgcactccagcctgggcaacaagagtgaaactccatctcaaaaaagaaaaaaaaaaaaaaaaggccgggcgtggtggctcacatctgtaatcctagcacttggggaggccgaggcaggcagattacctgagttcaggagttttagaacagcctgggcaacacggtgaaaccccgtctctactaaaatgcaaaaaattagctgggcgtggcagtgtgtgcctgcagtcccagctactcgggaggctgaggcaggataattgcttgcacccaggaggcagaggttgcagtgagccgagatcgtgccaccgcactccaccctgcgcgacagagcaaaactccgtctcaaaataaaaaaaaataaaaaataaaaaaatctgtgttaaataactaaagttgaaaattgaatgtcagttttattatggtggattttctcccgtgtcttcacgactcacagcgctgagtgtgctaaccaatggtgggcttaattggggtactaggctcaggaaatagctgccattcttgctaccaagtggcctcacataattatcttaaggcatctcttgagctgaaacaggtggggctggtaattggcagcctcaagtaaaataggaggagagagaggctcagagtgggttgcagaggaactggtgaataaattcttgagccttcttcttctctgtcatatcaagcttttggtgaccagctgggtttcgaagcaataagctgccaaatatgctagctagaatattctcatccaaatgattttttgctgaatttttcagcagttctcgcaaaaacgccatcaagtagtggaagacatttttgtggaatatggggagagtagaaatgacctgtttgcttgctgtgtagttgccagaacactccaagcagttatggtaggtgctgtaacagatgacaggctctggaaggctctccaggaaaagcagcagggcttcggctacagaatgattgctggcagagaggttatcaatcattccagtatccaagcagtccctgatatgttcaaattctgacctcaggcctggttgctgaaacagatcttcctgctggacagcatttcggtacaggtaatcaaccatcatccagagctctttggggatttccatggggctatccaactggctcccatcatctccagtccatactggcatcagagtcagctcactaatggtttcaagtggtaggtccaagattggctctctcatgtaacacagtgtatgaatgggagacccaaaacagctgggcaggtagttcccagacacagacaaaaagtaatcctttcccctgtccaagtgcagaaccagaatgtcctcaattttgtcttcacccgagttgagctttgtagctgtcatcttatttacgaagagctccaagtcaatctcaacatcagaatctggcaggaggaagcctctgctggggttggcattcagccactgcttacagtaagactcttcatcaggcttgttgatgaattcaaaatgacagggtacttgtccattatgaattgtaaaggattctactttcaattgcatgtacttcacattctgaaaacagaactctcgcttggacagggacacagaaggaatgttggcattttccatcttatccagggagcgaacaatttcctccagtgtcttccggtaaagctcgtcatttacgaccctcaccccgatgtcaaacactgagctgacaggcttgtggtcactggtcttcagggccatgtggctctggtaactcagctgagtgatgttcttccctttccagagaatccgatcacaccaggcaggagcacggcacttctcactgaaatgcaaagtccacactggaagtactcacagaaacagcagtgcccgctgcctggcgagtgccctggctcaggtggggagtgatgaatcagggccttcatgtccatgtggctaagtcatctgaggcagcaagagcaattcgggcccaccaagggataacatgtatcctgtgggtatcatccaaaacaaccatgaaagctcaaagccaaaacagagttcagactgattctctgatctttatcctcctggtatcccagtcgtcagagcccgtatcatacttgtaagtaggctggaatgtgagctcaccctctgtgaagccttcaaagacagtctttgcggccacctgaattttcagctgatcatatgcatacagcatttgaaagtccttctcttcgatgagctttttcactttttccacatccagctcttctatcctgtagttgaggtcccccagccacaagatcacatcatggttgctgatggtgagagggggaaggcttgggtcaggctgacaaaactgcattcgagaacaaatgtccttatagtcctggttcctcctctcatactcttcaatgtgggctgccaagtgagaattcacaacgcagatgctggtgttgtggaactggaacctgatcgccacgcctcccttgttgcccatcctccccatgattcctgtccccacagtctcggcttccacttctgagatataagctgcatgctcctgtttgacatataacagcagcataatcccaaccagtcggataagcttcacctttgcatatttggcatctggatgaagaccctctgacacagctttgaaccactcttcctcctttggggtatcgtgaaagaaaaaagcttccttactcagatcaagctcctggaaccctacacaatagacatctggggcctggataccattgctcagccacagccggaggcattctttgggggactgcccatttacattgtatgttcccgcaaaaaacctgaagttctggatataggtgtaatcctcttctttctgtagtagatgtgatttcacaattgtatctcgcagtccaaacttctgcatggataaaatatgagccttgtccgacactgtgatagtggaggagcgaaccatgtcagtaatttcggacttggatttattctgtcttggttgcaagctttctggtttatcttgacccctggagctttggtccataggcactcccttcccatttggtctcaaaccatcaaagttagaaccacctccgccaattgtcgcgtaccctggccaggtaactagggccgagttacaaccgcgcggcgttggcatctccagctccagctctgcgcacctataccgagacagccacaggaattcaggatcccgggtcgcagaatcgaagcctggacaggccctggcaacttcgtggaggaacatcctggtttgtgaaccaaagggcagttggaatacgaggctaagctctgctgtgtccagctggacggtcacatctgagccttgtccataaaatggagatgcaaacagtgataacctcatagagctgtgagaaaagcctgatttaggcccggtgcggtggctcatgcctgtaatcccagcactttgggaggccgaggtggggtggatcacaaggtcaggagatcgagaccatcctggccaacacggtgaaaccccgtctcaaggatgtagagttcaccatctggggacacttcttccagcgtaaaatcccgcgagactggcactatctggtccagagagacatcgtccccggtaatggccatcctccggtgcgtatagaggaagagagcgtgttcctggccgccgtgctccaggcggtagcgcacgagtcccaggaggcggctctgccggctgtccccctcacacagcacaccttgcaccgcgatgacgcagtattccccctcagccagcgtctcctggattgccacagactggtccatgctggcccctgctgagcgcacacaccctcctgagctgtcaccacagggcgcacgggactccgctgccccaggttccgggacagtgactacattt

SEQ ID NO: 18320 - RNA, 3419 nt, Homo sapiens
  source 1..3419: mol_type = other RNA
tgaagtaccagctactcgagaggctgaggcaggagaattgcttgaaccaaggaggcagaggttgcagtgagccaagaccacgccaacgcactccagcctgggcaacaagagtgaaactccatctcaaaaaagaaaaaaaaaaaaaaaaggccgggcgtggtggctcacatctgtaatcctagcacttggggaggccgaggcaggcagattacctgagttcaggagttttagaacagcctgggcaacacggtgaaaccccgtctctactaaaatgcaaaaaattagctgggcgtggcagtgtgtgcctgcagtcccagctactcgggaggctgaggcaggataattgcttgcacccaggaggcagaggttgcagtgagccgagatcgtgccaccgcactccaccctgcgcgacagagcaaaactccgtctcaaaataaaaaaaaataaaaaataaaaaaatctgtgttaaataactaaagttgaaaattgaatgtcagttttattatggtggattttctcccgtgtcttcacgactcacagcgctgagtgtgctaaccaatggtgggcttaattggggtactaggctcaggaaatagctgccattcttgctaccaagtggcctcacataattatcttaaggcatctcttgagctgaaacaggtggggctggtaattggcagcctcaagtaaaataggaggagagagaggctcagagtgggttgcagaggaactggtgaataaattcttgagccttcttcttctctgtcatatcaagcttttggtgaccagctgggtttcgaagcaataagctgccaaatatgctagctagaatattctcatccaaatgattttttgctgaatttttcagcagttctcgcaaaaacgccatcaagtagtggaagacatttttgtggaatatggggagagtagaaatgacctgtttgcttgctgtgtagttgccagaacactccaagcagttatggtaggtgctgtaacagatgacaggctctggaaggctctccaggaaaagcagcagggcttcggctacagaatgattgctggcagagaggttatcaatcattccagtatccaagcagtccctgatatgttcaaattctgacctcaggcctggttgctgaaacagatcttcctgctggacagcatttcggtacaggtaatcaaccatcatccagagctctttggggatttccatggggctatccaactggctcccatcatctccagtccatactggcatcagagtcagctcactaatggtttcaagtggtaggtccaagattggctctctcatgtaacacagtgtatgaatgggagacccaaaacagctgggcaggtagttcccagacacagacaaaaagtaatcctttcccctgtccaagtgcagaaccagaatgtcctcaattttgtcttcacccgagttgagctttgtagctgtcatcttatttacgaagagctccaagtcaatctcaacatcagaatctggcaggaggaagcctctgctggggttggcattcagccactgcttacagtaagactcttcatcaggcttgttgatgaattcaaaatgacagggtacttgtccattatgaattgtaaaggattctactttcaattgcatgtacttcacattctgaaaacagaactctcgcttggacagggacacagaaggaatgttggcattttccatcttatccagggagcgaacaatttcctccagtgtcttccggtaaagctcgtcatttacgaccctcaccccgatgtcaaacactgagctgacaggcttgtggtcactggtcttcagggccatgtggctctggtaactcagctgagtgatgttcttccctttccagagaatccgatcacaccaggcaggagcacggcacttctcactggtatcccagtcgtcagagcccgtatcatacttgtaagtaggctggaatgtgagctcaccctctgtgaagccttcaaagacagtctttgcggccacctgaattttcagctgatcatatgcatacagcatttgaaagtccttctcttcgatgagctttttcactttttccacatccagctcttctatcctgtagttgaggtcccccagccacaagatcacatcatggttgctgatggtgagagggggaaggcttgggtcaggctgacaaaactgcattcgagaacaaatgtccttatagtcctggttcctcctctcatactcttcaatgtgggctgccaagtgagaattcacaacgcagatgctggtgttgtggaactggaacctgatcgccacgcctcccttgttgcccatcctccccatgattcctgtccccacagtctcggcttccacttctgagatataagctgcatgctcctgtttgacatataacagcagcataatcccaaccagtcggataagcttcacctttgcatatttggcatctggatgaagaccctctgacacagctttgaaccactcttcctcctttggggtatcgtgaaagaaaaaagcttccttactcagatcaagctcctggaaccctacacaatagacatctggggcctggataccattgctcagccacagccggaggcattctttgggggactgcccatttacattgtatgttcccgcaaaaaacctgaagttctggatataggtgtaatcctcttctttctgtagtagatgtgatttcacaattgtatctcgcagtccaaacttctgcatggataaaatatgagccttgtccgacactgtgatagtggaggagcgaaccatgtcagtaatttcggacttggatttattctgtctcaggggcgagtcaggaaagagtaaataaaacaggaaaaaaagtcacttcagagtcaggaaacaccttggttgcaagctttctggtttatcttgacccctggagctttggtccataggcactcccttcccatttggtctcaaaccatcaaagttagaaccacctccgccaattgtcgcgtaccctggccaggtaactagggccgagttacaaccgcgcggcgttggcatctccagctccagctctgcgcacctataccgagacagccacaggaattcaggatcccgggtcgcagaatcgaagcctggacaggccctggcaacttcgtggaggaacatcctggtttgtgaaccaaagggcagttggaatacgaggctaagctctgctgtgtccagctggacggtcacatctgagccttgtccataaaatggagatgcaaacagtgataacctcatagagctgtgagaaaagcctgatttaggcccggtgcggtggctcatgcctgtaatcccagcactttgggaggccgaggtggggtggatcacaaggtcaggagatcgagaccatcctggccaacacggtgaaaccccgtctcta

SEQ ID NO: 18321 - RNA, 2973 nt, Homo sapiens
  source 1..2973: mol_type = other RNA
tgaagtaccagctactcgagaggctgaggcaggagaattgcttgaaccaaggaggcagaggttgcagtgagccaagaccacgccaacgcactccagcctgggcaacaagagtgaaactccatctcaaaaaagaaaaaaaaaaaaaaaaggccgggcgtggtggctcacatctgtaatcctagcacttggggaggccgaggcaggcagattacctgagttcaggagttttagaacagcctgggcaacacggtgaaaccccgtctctactaaaatgcaaaaaattagctgggcgtggcagtgtgtgcctgcagtcccagctactcgggaggctgaggcaggataattgcttgcacccaggaggcagaggttgcagtgagccgagatcgtgccaccgcactccaccctgcgcgacagagcaaaactccgtctcaaaataaaaaaaaataaaaaataaaaaaatctgtgttaaataactaaagttgaaaattgaatgtcagttttattatggtggattttctcccgtgtcttcacgactcacagcgctgagtgtgctaaccaatggtgggcttaattggggtactaggctcaggaaatagctgccattcttgctaccaagtggcctcacataattatcttaaggcatctcttgagctgaaacaggtggggctggtaattggcagcctcaagtaaaataggaggagagagaggctcagagtgggttgcagaggaactggtgaataaattcttgagccttcttcttctctgtcatatcaagcttttggtgaccagctgggtttcgaagcaataagctgccaaatatgctagctagaatattctcatccaaatgattttttgctgaatttttcagcagttctcgcaaaaacgccatcaagtagtggaagacatttttgtggaatatggggagagtagaaatgacctgtttgcttgctgtgtagttgccagaacactccaagcagttatggtaggtgctgtaacagatgacaggctctggaaggctctccaggaaaagcagcagggcttcggctacagaatgattgctggcagagaggttatcaatcattccagtatccaagcagtccctgatatgttcaaattctgacctcaggcctggttgctgaaacagatcttcctgctggacagcatttcggtacaggtaatcaaccatcatccagagctctttggggatttccatggggctatccaactggctcccatcatctccagtccatactggcatcagagtcagctcactaatggtttcaagtggtaggtccaagattggctctctcatgtaacacagtgtatgaatgggagacccaaaacagctgggcaggtagttcccagacacagacaaaaagtaatcctttcccctgtccaagtgcagaaccagaatgtcctcaattttgtcttcacccgagttgagctttgtagctgtcatcttatttacgaagagctccaagtcaatctcaacatcagaatctggcaggaggaagcctctgctggggttggcattcagccactgcttacagtaagactcttcatcaggcttgttgatgaattcaaaatgacagggtacttgtccattatgaattgtaaaggattctactttcaattgcatgtacttcacattctgaaaacagaactctcgcttggacagggacacagaaggaatgttggcattttccatcttatccagggagcgaacaatttcctccagtgtcttccggtaaagctcgtcatttacgaccctcaccccgatgtcaaacactgagctgacaggcttgtggtcactggtcttcagggccatgtggctctggtaactcagctgagtgatgttcttccctttccagagaatccgatcacaccaggcaggagcacggcacttctcactggtatcccagtcgtcagagcccgtatcatacttgtaagtaggctggaatgtgagctcaccctctgtgaagccttcaaagacagtctttgcggccacctgaattttcagctgatcatatgcatacagcatttgaaagtccttctcttcgatgagctttttcactttttccacatccagctcttctatcctgtagttgaggtcccccagccacaagatcacatcatggttgctgatggtgagagggggaaggcttgggtcaggctgacaaaactgcattcgagaacaaatgtccttatagtcctggttcctcctctcatactcttcaatgtgggctgccaagtgagaattcacaacgcagatgctggtgttgtggaactggaacctgatcgccacgcctcccttgttgcccatcctccccatgattcctgtccccacagtctcggcttccacttctgagatataagctgcatgctcctgtttgacatataacagcagcataatcccaaccagtcggataagcttcacctttgcatatttggcatctggatgaagaccctctgacacagctttgaaccactcttcctcctttggggtatcgtgaaagaaaaaagcttccttactcagatcaagctcctggaaccctacacaatagacatctggggcctggataccattgctcagccacagccggaggcattctttgggggactgcccatttacattgtatgttcccgcaaaaaacctgaagttctggatataggtgtaatcctcttctttctgtagtagatgtgatttcacaattgtatctcgcagtccaaacttctgcatggataaaatatgagccttgtccgacactgtgatagtggaggagcgaaccatgtcagtaatttcggacttggatttattctgtcttggttgcaagctttctggtttatcttgacccctggagctttggtccataggcactcccttcccatttggtctcaaaccatcaaagttagaaccaccctggccaggtaactagggccgagttacaaccgcgcggcgttggcatctccagc

SEQ ID NO: 18322 - RNA, 3539 nt, Homo sapiens
  source 1..3539: mol_type = other RNA
tgaagtaccagctactcgagaggctgaggcaggagaattgcttgaaccaaggaggcagaggttgcagtgagccaagaccacgccaacgcactccagcctgggcaacaagagtgaaactccatctcaaaaaagaaaaaaaaaaaaaaaaggccgggcgtggtggctcacatctgtaatcctagcacttggggaggccgaggcaggcagattacctgagttcaggagttttagaacagcctgggcaacacggtgaaaccccgtctctactaaaatgcaaaaaattagctgggcgtggcagtgtgtgcctgcagtcccagctactcgggaggctgaggcaggataattgcttgcacccaggaggcagaggttgcagtgagccgagatcgtgccaccgcactccaccctgcgcgacagagcaaaactccgtctcaaaataaaaaaaaataaaaaataaaaaaatctgtgttaaataactaaagttgaaaattgaatgtcagttttattatggtggattttctcccgtgtcttcacgactcacagcgctgagtgtgctaaccaatggtgggcttaattggggtactaggctcaggaaatagctgccattcttgctaccaagtggcctcacataattatcttaaggcatctcttgagctgaaacaggtggggctggtaattggcagcctcaagtaaaataggaggagagagaggctcagagtgggttgcagaggaactggtgaataaattcttgagccttcttcttctctgtcatatcaagcttttggtgaccagctgggtttcgaagcaataagctgccaaatatgctagctagaatattctcatccaaatgattttttgctgaatttttcagcagttctcgcaaaaacgccatcaagtagtggaagacatttttgtggaatatggggagagtagaaatgacctgtttgcttgctgtgtagttgccagaacactccaagcagttatggtaggtgctgtaacagatgacaggctctggaaggctctccaggaaaagcagcagggcttcggctacagaatgattgctggcagagaggttatcaatcattccagtatccaagcagtccctgatatgttcaaattctgacctcaggcctggttgctgaaacagatcttcctgctggacagcatttcggtacaggtaatcaaccatcatccagagctctttggggatttccatggggctatccaactggctcccatcatctccagtccatactggcatcagagtcagctcactaatggtttcaagtggtaggtccaagattggctctctcatgtaacacagtgtatgaatgggagacccaaaacagctgggcaggtagttcccagacacagacaaaaagtaatcctttcccctgtccaagtgcagaaccagaatgtcctcaattttgtcttcacccgagttgagctttgtagctgtcatcttatttacgaagagctccaagtcaatctcaacatcagaatctggcaggaggaagcctctgctggggttggcattcagccactgcttacagtaagactcttcatcaggcttgttgatgaattcaaaatgacagggtacttgtccattatgaattgtaaaggattctactttcaattgcatgtacttcacattctgaaaacagaactctcgcttggacagggacacagaaggaatgttggcattttccatcttatccagggagcgaacaatttcctccagtgtcttccggtaaagctcgtcatttacgaccctcaccccgatgtcaaacactgagctgacaggcttgtggtcactggtcttcagggccatgtggctctggtaactcagctgagtgatgttcttccctttccagagaatccgatcacaccaggcaggagcacggcacttctcactggtatcccagtcgtcagagcccgtatcatacttgtaagtaggctggaatgtgagctcaccctctgtgaagccttcaaagacagtctttgcggccacctgaattttcagctgatcatatgcatacagcatttgaaagtccttctcttcgatgagctttttcactttttccacatccagctcttctatcctgtagttgaggtcccccagccacaagatcacatcatggttgctgatggtgagagggggaaggcttgggtcaggctgacaaaactgcattcgagaacaaatgtccttatagtcctggttcctcctctcatactcttcaatgtgggctgccaagtgagaattcacaacgcagatgctggtgttgtggaactggaacctgatcgccacgcctcccttgttgcccatcctccccatgattcctgtccccacagtctcggcttccacttctgagatataagctgcatgctcctgtttgacatataacagcagcataatcccaaccagtcggataagcttcacctttgcatatttggcatctggatgaagaccctctgacacagctttgaaccactcttcctcctttggggtatcgtgaaagaaaaaagcttccttactcagatcaagctcctggaaccctacacaatagacatctggggcctggataccattgctcagccacagccggaggcattctttgggggactgcccatttacattgtatgttcccgcaaaaaacctgaagttctggatataggtgtaatcctcttctttctgtagtagatgtgatttcacaattgtatctcgcagtccaaacttctgcatggataaaatatgagccttgtccgacactgtgatagtggaggagcgaaccatgtcagtaatttcggacttggatttattctgtcttggttgcaagctttctggtttatcttgacccctggagctttggtccataggcactcccttcccatttggtctcaaaccatcaaagttagaaccacctccgccaattgtcgcgtaccctggccaggtaactagggccgagttacaaccgcgcggcgttggcatctccagctccagctctgcgcacctataccgagacagccacaggaattcaggatcccgggtcgcagaatcgaagcctggacaggccctggcaacttcgtggaggaacatcctggtttgtgaaccaaagggcagttggaatacgaggctaagctctgctgtgtccagctggacggtcacatcaaggatgtagagttcaccatctggggacacttcttccagcgtaaaatcccgcgagactggcactatctggtccagagagacatcgtccccggtaatggccatcctccggtgcgtatagaggaagagagcgtgttcctggccgccgtgctccaggcggtagcgcacgagtcccaggaggcggctctgccggctgtccccctcacacagcacaccttgcaccgcgatgacgcagtattccccctcagccagcgtctcctggattgccacagactggtccatgctggcccctgctgagcgcacacaccctcctgagctgtcaccacagggcgcacgggactccgctgccccaggttccgggacagtgactacattt

SEQ ID NO: 18323 - RNA, 3541 nt, Homo sapiens
  source 1..3541: mol_type = other RNA
tgaagtaccagctactcgagaggctgaggcaggagaattgcttgaaccaaggaggcagaggttgcagtgagccaagaccacgccaacgcactccagcctgggcaacaagagtgaaactccatctcaaaaaagaaaaaaaaaaaaaaaaggccgggcgtggtggctcacatctgtaatcctagcacttggggaggccgaggcaggcagattacctgagttcaggagttttagaacagcctgggcaacacggtgaaaccccgtctctactaaaatgcaaaaaattagctgggcgtggcagtgtgtgcctgcagtcccagctactcgggaggctgaggcaggataattgcttgcacccaggaggcagaggttgcagtgagccgagatcgtgccaccgcactccaccctgcgcgacagagcaaaactccgtctcaaaataaaaaaaaataaaaaataaaaaaatctgtgttaaataactaaagttgaaaattgaatgtcagttttattatggtggattttctcccgtgtcttcacgactcacagcgctgagtgtgctaaccaatggtgggcttaattggggtactaggctcaggaaatagctgccattcttgctaccaagtggcctcacataattatcttaaggcatctcttgagctgaaacaggtggggctggtaattggcagcctcaagtaaaataggaggagagagaggctcagagtgggttgcagaggaactggtgaataaattcttgagccttcttcttctctgtcatatcaagcttttggtgaccagctgggtttcgaagcaataagctgccaaatatgctagctagaatattctcatccaaatgattttttgctgaatttttcagcagttctcgcaaaaacgccatcaagtagtggaagacatttttgtggaatatggggagagtagaaatgacctgtttgcttgctgtgtagttgccagaacactccaagcagttatggtaggtgctgtaacagatgacaggctctggaaggctctccaggaaaagcagcagggcttcggctacagaatgattgctggcagagaggttatcaatcattccagtatccaagcagtccctgatatgttcaaattctgacctcaggcctggttgctgaaacagatcttcctgctggacagcatttcggtacaggtaatcaaccatcatccagagctctttggggatttccatggggctatccaactggctcccatcatctccagtccatactggcatcagagtcagctcactaatggtttcaagtggtaggtccaagattggctctctcatgtaacacagtgtatgaatgggagacccaaaacagctgggcaggtagttcccagacacagacaaaaagtaatcctttcccctgtccaagtgcagaaccagaatgtcctcaattttgtcttcacccgagttgagctttgtagctgtcatcttatttacgaagagctccaagtcaatctcaacatcagaatctggcaggaggaagcctctgctggggttggcattcagccactgcttacagtaagactcttcatcaggcttgttgatgaattcaaaatgacagggtacttgtccattatgaattgtaaaggattctactttcaattgcatgtacttcacattctgaaaacagaactctcgcttggacagggacacagaaggaatgttggcattttccatcttatccagggagcgaacaatttcctccagtgtcttccggtaaagctcgtcatttacgaccctcaccccgatgtcaaacactgagctgacaggcttgtggtcactggtcttcagggccatgtggctctggtaactcagctgagtgatgttcttccctttccagagaatccgatcacaccaggcaggagcacggcacttctcactggtatcccagtcgtcagagcccgtatcatacttgtaagtaggctggaatgtgagctcaccctctgtgaagccttcaaagacagtctttgcggccacctgaattttcagctgatcatatgcatacagcatttgaaagtccttctcttcgatgagctttttcactttttccacatccagctcttctatcctgtagttgaggtcccccagccacaagatcacatcatggttgctgatggtgagagggggaaggcttgggtcaggctgacaaaactgcattcgagaacaaatgtccttatagtcctggttcctcctctcatactcttcaatgtgggctgccaagtgagaattcacaacgcagatgctggtgttgtggaactggaacctgatcgccacgcctcccttgttgcccatcctccccatgattcctgtccccacagtctcggcttccacttctgagatataagctgcatgctcctgtttgacatataacagcagcataatcccaaccagtcggataagcttcacctttgcatatttggcatctggatgaagaccctctgacacagctttgaaccactcttcctcctttggggtatcgtgaaagaaaaaagcttccttactcagatcaagctcctggaaccctacacaatagacatctggggcctggataccattgctcagccacagccggaggcattctttgggggactgcccatttacattgtatgttcccgcaaaaaacctgaagttctggatataggtgtaatcctcttctttctgtagtagatgtgatttcacaattgtatctcgcagtccaaacttctgcatggataaaatatgagccttgtccgacactgtgatagtggaggagcgaaccatgtcagtaatttcggacttggatttattctgtcttggttgcaagctttctggtttatcttgacccctggagctttggtccataggcactcccttcccatttggtctcaaaccatcaaagttagaaccacctccgccaattgtcgcgtaccctggccaggtaactagggccgagttacaaccgcgcggcgttggcatctccagctccagctctgcgcacctataccgagacagccacaggaattcaggatcccgggtcgcagaatcgaagcctggacaggccctggcaacttcgtggaggaacatcctggtttgtgaaccaaagggcagttggaatacgaggctaagctctgctgtgtccagctggacggtcacatctgagccaaggatgtagagttcaccatctggggacacttcttccagcgtaaaatcccgcgagactggcactatctggtccagagagacatcgtccccggtaatggccatcctccggtgcgtatagaggaagagagcgtgttcctggccgccgtgctccaggcggtagcgcacgagtcccaggaggcggctctgccggctgtccccctcacacagcacaccttgcaccgcgatgacgcagtattccccctcagccagcgtctcctggattgccacagactggtccatgctggcccctgctgagcgcacacaccctcctgagctgtcaccacagggcgcacgggactccgctgccccaggttccgggacagtgactac

SEQ ID NO: 18324 - RNA, 3573 nt, Homo sapiens
  source 1..3573: mol_type = other RNA
tgaagtaccagctactcgagaggctgaggcaggagaattgcttgaaccaaggaggcagaggttgcagtgagccaagaccacgccaacgcactccagcctgggcaacaagagtgaaactccatctcaaaaaagaaaaaaaaaaaaaaaaggccgggcgtggtggctcacatctgtaatcctagcacttggggaggccgaggcaggcagattacctgagttcaggagttttagaacagcctgggcaacacggtgaaaccccgtctctactaaaatgcaaaaaattagctgggcgtggcagtgtgtgcctgcagtcccagctactcgggaggctgaggcaggataattgcttgcacccaggaggcagaggttgcagtgagccgagatcgtgccaccgcactccaccctgcgcgacagagcaaaactccgtctcaaaataaaaaaaaataaaaaataaaaaaatctgtgttaaataactaaagttgaaaattgaatgtcagttttattatggtggattttctcccgtgtcttcacgactcacagcgctgagtgtgctaaccaatggtgggcttaattggggtactaggctcaggaaatagctgccattcttgctaccaagtggcctcacataattatcttaaggcatctcttgagctgaaacaggtggggctggtaattggcagcctcaagtaaaataggaggagagagaggctcagagtgggttgcagaggaactggtgaataaattcttgagccttcttcttctctgtcatatcaagcttttggtgaccagctgggtttcgaagcaataagctgccaaatatgctagctagaatattctcatccaaatgattttttgctgaatttttcagcagttctcgcaaaaacgccatcaagtagtggaagacatttttgtggaatatggggagagtagaaatgacctgtttgcttgctgtgtagttgccagaacactccaagcagttatggtaggtgctgtaacagatgacaggctctggaaggctctccaggaaaagcagcagggcttcggctacagaatgattgctggcagagaggttatcaatcattccagtatccaagcagtccctgatatgttcaaattctgacctcaggcctggttgctgaaacagatcttcctgctggacagcatttcggtacaggtaatcaaccatcatccagagctctttggggatttccatggggctatccaactggctcccatcatctccagtccatactggcatcagagtcagctcactaatggtttcaagtggtaggtccaagattggctctctcatgtaacacagtgtatgaatgggagacccaaaacagctgggcaggtagttcccagacacagacaaaaagtaatcctttcccctgtccaagtgcagaaccagaatgtcctcaattttgtcttcacccgagttgagctttgtagctgtcatcttatttacgaagagctccaagtcaatctcaacatcagaatctggcaggaggaagcctctgctggggttggcattcagccactgcttacagtaagactcttcatcaggcttgttgatgaattcaaaatgacagggtacttgtccattatgaattgtaaaggattctactttcaattgcatgtacttcacattctgaaaacagaactctcgcttggacagggacacagaaggaatgttggcattttccatcttatccagggagcgaacaatttcctccagtgtcttccggtaaagctcgtcatttacgaccctcaccccgatgtcaaacactgagctgacaggcttgtggtcactggtcttcagggccatgtggctctggtaactcagctgagtgatgttcttccctttccagagaatccgatcacaccaggcaggagcacggcacttctcactggtatcccagtcgtcagagcccgtatcatacttgtaagtaggctggaatgtgagctcaccctctgtgaagccttcaaagacagtctttgcggccacctgaattttcagctgatcatatgcatacagcatttgaaagtccttctcttcgatgagctttttcactttttccacatccagctcttctatcctgtagttgaggtcccccagccacaagatcacatcatggttgctgatggtgagagggggaaggcttgggtcaggctgacaaaactgcattcgagaacaaatgtccttatagtcctggttcctcctctcatactcttcaatgtgggctgccaagtgagaattcacaacgcagatgctggtgttgtggaactggaacctgatcgccacgcctcccttgttgcccatcctccccatgattcctgtccccacagtctcggcttccacttctgagatataagctgcatgctcctgtttgacatataacagcagcataatcccaaccagtcggataagcttcacctttgcatatttggcatctggatgaagaccctctgacacagctttgaaccactcttcctcctttggggtatcgtgaaagaaaaaagcttccttactcagatcaagctcctggaaccctacacaatagacatctggggcctggataccattgctcagccacagccggaggcattctttgggggactgcccatttacattgtatgttcccgcaaaaaacctgaagttctggatataggtgtaatcctcttctttctgtagtagatgtgatttcacaattgtatctcgcagtccaaacttctgcatggataaaatatgagccttgtccgacactgtgatagtggaggagcgaaccatgtcagtaatttcggacttggatttattctgtcttggttgcaagctttctggtttatcttgacccctggagctttggtccataggcactcccttcccatttggtctcaaaccatcaaagttagaaccacctccgccaattgtcgcgtaccctggccaggtaactagggccgagttacaaccgcgcggcgttggcatctccagctccagctctgcgcacctataccgagacagccacaggaattcaggatcccgggtcgcagaatcgaagcctggacaggccctggcaacttcgtggaggaacatcctggtttgtgaaccaaagggcagttggaatacgaggctaagctctgctgtgtccagctggacggtcacatctgagccaaggatgtagagttcaccatctggggacacttcttccagcgtaaaatcccgcgagactggcactatctggtccagagagacatcgtccccggtaatggccatcctccggtgcgtatagaggaagagagcgtgttcctggccgccgtgctccaggcggtagcgcacgagtcccaggaggcggctctgccggctgtccccctcacacagcacaccttgcaccgcgatgacgcagtattccccctcagccagcgtctcctggattgccacagactggtccatgctggcccctgctgagcgcacacacctgtcattcaggagggtcccattcctctttccttggagacaggaagtgtcccattgctgcttgcccttcacccccgccccagcaggcccattgcatc

SEQ ID NO: 18325 - RNA, 3447 nt, Homo sapiens
  source 1..3447: mol_type = other RNA
tgaagtaccagctactcgagaggctgaggcaggagaattgcttgaaccaaggaggcagaggttgcagtgagccaagaccacgccaacgcactccagcctgggcaacaagagtgaaactccatctcaaaaaagaaaaaaaaaaaaaaaaggccgggcgtggtggctcacatctgtaatcctagcacttggggaggccgaggcaggcagattacctgagttcaggagttttagaacagcctgggcaacacggtgaaaccccgtctctactaaaatgcaaaaaattagctgggcgtggcagtgtgtgcctgcagtcccagctactcgggaggctgaggcaggataattgcttgcacccaggaggcagaggttgcagtgagccgagatcgtgccaccgcactccaccctgcgcgacagagcaaaactccgtctcaaaataaaaaaaaataaaaaataaaaaaatctgtgttaaataactaaagttgaaaattgaatgtcagttttattatggtggattttctcccgtgtcttcacgactcacagcgctgagtgtgctaaccaatggtgggcttaattggggtactaggctcaggaaatagctgccattcttgctaccaagtggcctcacataattatcttaaggcatctcttgagctgaaacaggtggggctggtaattggcagcctcaagtaaaataggaggagagagaggctcagagtgggttgcagaggaactggtgaataaattcttgagccttcttcttctctgtcatatcaagcttttggtgaccagctgggtttcgaagcaataagctgccaaatatgctagctagaatattctcatccaaatgattttttgctgaatttttcagcagttctcgcaaaaacgccatcaagtagtggaagacatttttgtggaatatggggagagtagaaatgacctgtttgcttgctgtgtagttgccagaacactccaagcagttatggtaggtgctgtaacagatgacaggctctggaaggctctccaggaaaagcagcagggcttcggctacagaatgattgctggcagagaggttatcaatcattccagtatccaagcagtccctgatatgttcaaattctgacctcaggcctggttgctgaaacagatcttcctgctggacagcatttcggtacaggtaatcaaccatcatccagagctctttggggatttccatggggctatccaactggctcccatcatctccagtccatactggcatcagagtcagctcactaatggtttcaagtggtaggtccaagattggctctctcatgtaacacagtgtatgaatgggagacccaaaacagctgggcaggtagttcccagacacagacaaaaagtaatcctttcccctgtccaagtgcagaaccagaatgtcctcaattttgtcttcacccgagttgagctttgtagctgtcatcttatttacgaagagctccaagtcaatctcaacatcagaatctggcaggaggaagcctctgctggggttggcattcagccactgcttacagtaagactcttcatcaggcttgttgatgaattcaaaatgacagggtacttgtccattatgaattgtaaaggattctactttcaattgcatgtacttcacattctgaaaacagaactctcgcttggacagggacacagaaggaatgttggcattttccatcttatccagggagcgaacaatttcctccagtgtcttccggtaaagctcgtcatttacgaccctcaccccgatgtcaaacactgagctgacaggcttgtggtcactggtcttcagggccatgtggctctggtaactcagctgagtgatgttcttccctttccagagaatccgatcacaccaggcaggagcacggcacttctcactggtatcccagtcgtcagagcccgtatcatacttgtaagtaggctggaatgtgagctcaccctctgtgaagccttcaaagacagtctttgcggccacctgaattttcagctgatcatatgcatacagcatttgaaagtccttctcttcgatgagctttttcactttttccacatccagctcttctatcctgtagttgaggtcccccagccacaagatcacatcatggttgctgatggtgagagggggaaggcttgggtcaggctgacaaaactgcattcgagaacaaatgtccttatagtcctggttcctcctctcatactcttcaatgtgggctgccaagtgagaattcacaacgcagatgctggtgttgtggaactggaacctgatcgccacgcctcccttgttgcccatcctccccatgattcctgtccccacagtctcggcttccacttctgagatataagctgcatgctcctgtttgacatataacagcagcataatcccaaccagtcggataagcttcacctttgcatatttggcatctggatgaagaccctctgacacagctttgaaccactcttcctcctttggggtatcgtgaaagaaaaaagcttccttactcagatcaagctcctggaaccctacacaatagacatctggggcctggataccattgctcagccacagccggaggcattctttgggggactgcccatttacattgtatgttcccgcaaaaaacctgaagttctggatataggtgtaatcctcttctttctgtagtagatgtgatttcacaattgtatctcgcagtccaaacttctgcatggataaaatatgagccttgtccgacactgtgatagtggaggagcgaaccatgtcagtaatttcggacttggatttattctgtcttggttgcaagctttctggtttatcttgacccctggagctttggtccataggcactcccttcccatttggtctcaaaccatcaaagttagaaccacctccgccaattgtcgcgtaccctggccaggtaactagggccgagttacaaccgcgcggcgttggcatctccagctccagctctgcgcacctataccgagacagccacaggaattcaggatcccgggtcgcagaatcgaagcctggacaggccctggcaacttcgtggaggaacatcctggtttgtgaaccaaagggcagttggaatacgaggctaagctctgctgtgtccagctggacggtcacatctgagccaaggatgtagagttcaccatctggggacagcgtgttcctggccgccgtgctccaggcggtagcgcacgagtcccaggaggcggctctgccggctgtccccctcacacagcacaccttgcaccgcgatgacgcagtattccccctcagccagcgtctcctggattgccacagactggtccatgctggcccctgctgagcgcacacaccctcctgagctgtcaccacagggcgcacgggactccgctgccccaggttccgggacagtgactacattt

SEQ ID NO: 18326 - RNA, 3475 nt, Homo sapiens
  source 1..3475: mol_type = other RNA
tgaagtaccagctactcgagaggctgaggcaggagaattgcttgaaccaaggaggcagaggttgcagtgagccaagaccacgccaacgcactccagcctgggcaacaagagtgaaactccatctcaaaaaagaaaaaaaaaaaaaaaaggccgggcgtggtggctcacatctgtaatcctagcacttggggaggccgaggcaggcagattacctgagttcaggagttttagaacagcctgggcaacacggtgaaaccccgtctctactaaaatgcaaaaaattagctgggcgtggcagtgtgtgcctgcagtcccagctactcgggaggctgaggcaggataattgcttgcacccaggaggcagaggttgcagtgagccgagatcgtgccaccgcactccaccctgcgcgacagagcaaaactccgtctcaaaataaaaaaaaataaaaaataaaaaaatctgtgttaaataactaaagttgaaaattgaatgtcagttttattatggtggattttctcccgtgtcttcacgactcacagcgctgagtgtgctaaccaatggtgggcttaattggggtactaggctcaggaaatagctgccattcttgctaccaagtggcctcacataattatcttaaggcatctcttgagctgaaacaggtggggctggtaattggcagcctcaagtaaaataggaggagagagaggctcagagtgggttgcagaggaactggtgaataaattcttgagccttcttcttctctgtcatatcaagcttttggtgaccagctgggtttcgaagcaataagctgccaaatatgctagctagaatattctcatccaaatgattttttgctgaatttttcagcagttctcgcaaaaacgccatcaagtagtggaagacatttttgtggaatatggggagagtagaaatgacctgtttgcttgctgtgtagttgccagaacactccaagcagttatggtaggtgctgtaacagatgacaggctctggaaggctctccaggaaaagcagcagggcttcggctacagaatgattgctggcagagaggttatcaatcattccagtatccaagcagtccctgatatgttcaaattctgacctcaggcctggttgctgaaacagatcttcctgctggacagcatttcggtacaggtaatcaaccatcatccagagctctttggggatttccatggggctatccaactggctcccatcatctccagtccatactggcatcagagtcagctcactaatggtttcaagtggtaggtccaagattggctctctcatgtaacacagtgtatgaatgggagacccaaaacagctgggcaggtagttcccagacacagacaaaaagtaatcctttcccctgtccaagtgcagaaccagaatgtcctcaattttgtcttcacccgagttgagctttgtagctgtcatcttatttacgaagagctccaagtcaatctcaacatcagaatctggcaggaggaagcctctgctggggttggcattcagccactgcttacagtaagactcttcatcaggcttgttgatgaattcaaaatgacagggtacttgtccattatgaattgtaaaggattctactttcaattgcatgtacttcacattctgaaaacagaactctcgcttggacagggacacagaaggaatgttggcattttccatcttatccagggagcgaacaatttcctccagtgtcttccggtaaagctcgtcatttacgaccctcaccccgatgtcaaacactgagctgacaggcttgtggtcactggtcttcagggccatgtggctctggtaactcagctgagtgatgttcttccctttccagagaatccgatcacaccaggcaggagcacggcacttctcactggtatcccagtcgtcagagcccgtatcatacttgtaagtaggctggaatgtgagctcaccctctgtgaagccttcaaagacagtctttgcggccacctgaattttcagctgatcatatgcatacagcatttgaaagtccttctcttcgatgagctttttcactttttccacatccagctcttctatcctgtagttgaggtcccccagccacaagatcacatcatggttgctgatggtgagagggggaaggcttgggtcaggctgacaaaactgcattcgagaacaaatgtccttatagtcctggttcctcctctcatactcttcaatgtgggctgccaagtgagaattcacaacgcagatgctggtgttgtggaactggaacctgatcgccacgcctcccttgttgcccatcctccccatgattcctgtccccacagtctcggcttccacttctgagatataagctgcatgctcctgtttgacatataacagcagcataatcccaaccagtcggataagcttcacctttgcatatttggcatctggatgaagaccctctgacacagctttgaaccactcttcctcctttggggtatcgtgaaagaaaaaagcttccttactcagatcaagctcctggaaccctacacaatagacatctggggcctggataccattgctcagccacagccggaggcattctttgggggactgcccatttacattgtatgttcccgcaaaaaacctgaagttctggatataggtgtaatcctcttctttctgtagtagatgtgatttcacaattgtatctcgcagtccaaacttctgcatggataaaatatgagccttgtccgacactgtgatagtggaggagcgaaccatgtcagtaatttcggacttggatttattctgtcttggttgcaagctttctggtttatcttgacccctggagctttggtccataggcactcccttcccatttggtctcaaaccatcaaagttagaaccacctccgccaattgtcgcgtaccctggccaggtaactagggccgagttacaaccgcgcggcgttggcatctccagctccagctctgcgcacctataccgagacagccacaggaattcaggatcccgggtcgcagaatcgaagcctggacaggccctggcaacttcgtggaggaacatcctggtttgtgaaccaaagggcagttggaatacgaggctaagctctgctgtgtccagctggacggtcacatctgagccaaggatgtagagttcaccatctggggacagcgtgttcctggccgccgtgctccaggcggtagcgcacgagtcccaggaggcggctctgccggctgtccccctcacacagcacaccttgcaccgcgatgacgcagtattccccctcagccagcgtctcctggattgccacagactggtccatgctggcccctgctgagcgcacacacctgtcattcaggagggtcccattcctctttccttggagacaggaagtgtcccattgctgcttgcccttcacccccgccccagcaggcccattgcatc

SEQ ID NO: 18327 - RNA, 3724 nt, Homo sapiens
  source 1..3724: mol_type = other RNA
tgaagtaccagctactcgagaggctgaggcaggagaattgcttgaaccaaggaggcagaggttgcagtgagccaagaccacgccaacgcactccagcctgggcaacaagagtgaaactccatctcaaaaaagaaaaaaaaaaaaaaaaggccgggcgtggtggctcacatctgtaatcctagcacttggggaggccgaggcaggcagattacctgagttcaggagttttagaacagcctgggcaacacggtgaaaccccgtctctactaaaatgcaaaaaattagctgggcgtggcagtgtgtgcctgcagtcccagctactcgggaggctgaggcaggataattgcttgcacccaggaggcagaggttgcagtgagccgagatcgtgccaccgcactccaccctgcgcgacagagcaaaactccgtctcaaaataaaaaaaaataaaaaataaaaaaatctgtgttaaataactaaagttgaaaattgaatgtcagttttattatggtggattttctcccgtgtcttcacgactcacagcgctgagtgtgctaaccaatggtgggcttaattggggtactaggctcaggaaatagctgccattcttgctaccaagtggcctcacataattatcttaaggcatctcttgagctgaaacaggtggggctggtaattggcagcctcaagtaaaataggaggagagagaggctcagagtgggttgcagaggaactggtgaataaattcttgagccttcttcttctctgtcatatcaagcttttggtgaccagctgggtttcgaagcaataagctgccaaatatgctagctagaatattctcatccaaatgattttttgctgaatttttcagcagttctcgcaaaaacgccatcaagtagtggaagacatttttgtggaatatggggagagtagaaatgacctgtttgcttgctgtgtagttgccagaacactccaagcagttatggtaggtgctgtaacagatgacaggctctggaaggctctccaggaaaagcagcagggcttcggctacagaatgattgctggcagagaggttatcaatcattccagtatccaagcagtccctgatatgttcaaattctgacctcaggcctggttgctgaaacagatcttcctgctggacagcatttcggtacaggtaatcaaccatcatccagagctctttggggatttccatggggctatccaactggctcccatcatctccagtccatactggcatcagagtcagctcactaatggtttcaagtggtaggtccaagattggctctctcatgtaacacagtgtatgaatgggagacccaaaacagctgggcaggtagttcccagacacagacaaaaagtaatcctttcccctgtccaagtgcagaaccagaatgtcctcaattttgtcttcacccgagttgagctttgtagctgtcatcttatttacgaagagctccaagtcaatctcaacatcagaatctggcaggaggaagcctctgctggggttggcattcagccactgcttacagtaagactcttcatcaggcttgttgatgaattcaaaatgacagggtacttgtccattatgaattgtaaaggattctactttcaattgcatgtacttcacattctgaaaacagaactctcgcttggacagggacacagaaggaatgttggcattttccatcttatccagggagcgaacaatttcctccagtgtcttccggtaaagctcgtcatttacgaccctcaccccgatgtcaaacactgagctgacaggcttgtggtcactggtcttcagggccatgtggctctggtaactcagctgagtgatgttcttccctttccagagaatccgatcacaccaggcaggagcacggcacttctcactggtatcccagtcgtcagagcccgtatcatacttgtaagtaggctggaatgtgagctcaccctctgtgaagccttcaaagacagtctttgcggccacctgaattttcagctgatcatatgcatacagcatttgaaagtccttctcttcgatgagctttttcactttttccacatccagctcttctatcctgtagttgaggtcccccagccacaagatcacatcatggttgctgatggtgagagggggaaggcttgggtcaggctgacaaaactgcattcgagaacaaatgtccttatagtcctggttcctcctctcatactcttcaatgtgggctgccaagtgagaattcacaacgcagatgctggtgttgtggaactggaacctgatcgccacgcctcccttgttgcccatcctccccatgattcctgtccccacagtctcggcttccacttctgagatataagctgcatgctcctgtttgacatataacagcagcataatcccaaccagtcggataagcttcacctttgcatatttggcatctggatgaagaccctctgacacagctttgaaccactcttcctcctttggggtatcgtgaaagaaaaaagcttccttactcagatcaagctcctggaaccctacacaatagacatctggggcctggataccattgctcagccacagccggaggcattctttgggggactgcccatttacattgtatgttcccgcaaaaaacctgaagttctggatataggtgtaatcctcttctttctgtagtagatgtgatttcacaattgtatctcgcagtccaaacttctgcatggataaaatatgagccttgtccgacactgtgatagtggaggagcgaaccatgtcagtaatttcggacttggatttattctgtcttggttgcaagctttctggtttatcttgacccctggagctttggtccataggcactcccttcccatttggtctcaaaccatcaaagttagaaccacctccgccaattgtcgcgtaccctggccaggtaactagggccgagttacaaccgcgcggcgttggcatctccagctccagctctgcgcacctataccgagacagccacaggaattcaggatcccgggtcgcagaatcgaagcctggacaggccctggcaacttcgtggaggaacatcctggtttgtgaaccaaagggcagttggaatacgaggctaagctctgctgtgtccagctggacggtcacatctgagccttgtccataaaatggagatgcaaacagtgataacctcatagagctgtgagaaaagcctgatttaggcccggtgcggtggctcatgcctgtaatcccagcactttgggaggccgaggtggggtggatcacaaggtcaggagatcgagaccatcctggccaacacggtgaaaccccgtctcaaggatgtagagttcaccatctggggacacttcttccagcgtaaaatcccgcgagactggcactatctggtccagagagacatcgtccccggtaatggccatcctccggtgcgtatagaggaagagagcgtgttcctggccgccgtgctccaggcggtagcgcacgagtcccaggaggcggctctgccggctgtccccctcacacagcacaccttgcaccgcgatgacgcagtattccccctcagccagcgtctcctggattgccacagactggtccatgctggcccctgctgagcgcacacaccctcctgagctgtcaccacagggcgcacgggactccgctgccccaggttccgggacagtgactacattt

SEQ ID NO: 18328 - RNA, 3727 nt, Homo sapiens
  source 1..3727: mol_type = other RNA
tgaagtaccagctactcgagaggctgaggcaggagaattgcttgaaccaaggaggcagaggttgcagtgagccaagaccacgccaacgcactccagcctgggcaacaagagtgaaactccatctcaaaaaagaaaaaaaaaaaaaaaaggccgggcgtggtggctcacatctgtaatcctagcacttggggaggccgaggcaggcagattacctgagttcaggagttttagaacagcctgggcaacacggtgaaaccccgtctctactaaaatgcaaaaaattagctgggcgtggcagtgtgtgcctgcagtcccagctactcgggaggctgaggcaggataattgcttgcacccaggaggcagaggttgcagtgagccgagatcgtgccaccgcactccaccctgcgcgacagagcaaaactccgtctcaaaataaaaaaaaataaaaaataaaaaaatctgtgttaaataactaaagttgaaaattgaatgtcagttttattatggtggattttctcccgtgtcttcacgactcacagcgctgagtgtgctaaccaatggtgggcttaattggggtactaggctcaggaaatagctgccattcttgctaccaagtggcctcacataattatcttaaggcatctcttgagctgaaacaggtggggctggtaattggcagcctcaagtaaaataggaggagagagaggctcagagtgggttgcagaggaactggtgaataaattcttgagccttcttcttctctgtcatatcaagcttttggtgaccagctgggtttcgaagcaataagctgccaaatatgctagctagaatattctcatccaaatgattttttgctgaatttttcagcagttctcgcaaaaacgccatcaagtagtggaagacatttttgtggaatatggggagagtagaaatgacctgtttgcttgctgtgtagttgccagaacactccaagcagttatggtaggtgctgtaacagatgacaggctctggaaggctctccaggaaaagcagcagggcttcggctacagaatgattgctggcagagaggttatcaatcattccagtatccaagcagtccctgatatgttcaaattctgacctcaggcctggttgctgaaacagatcttcctgctggacagcatttcggtacaggtaatcaaccatcatccagagctctttggggatttccatggggctatccaactggctcccatcatctccagtccatactggcatcagagtcagctcactaatggtttcaagtggtaggtccaagattggctctctcatgtaacacagtgtatgaatgggagacccaaaacagctgggcaggtagttcccagacacagacaaaaagtaatcctttcccctgtccaagtgcagaaccagaatgtcctcaattttgtcttcacccgagttgagctttgtagctgtcatcttatttacgaagagctccaagtcaatctcaacatcagaatctggcaggaggaagcctctgctggggttggcattcagccactgcttacagtaagactcttcatcaggcttgttgatgaattcaaaatgacagggtacttgtccattatgaattgtaaaggattctactttcaattgcatgtacttcacattctgaaaacagaactctcgcttggacagggacacagaaggaatgttggcattttccatcttatccagggagcgaacaatttcctccagtgtcttccggtaaagctcgtcatttacgaccctcaccccgatgtcaaacactgagctgacaggcttgtggtcactggtcttcagggccatgtggctctggtaactcagctgagtgatgttcttccctttccagagaatccgatcacaccaggcaggagcacggcacttctcactggtatcccagtcgtcagagcccgtatcatacttgtaagtaggctggaatgtgagctcaccctctgtgaagccttcaaagacagtctttgcggccacctgaattttcagctgatcatatgcatacagcatttgaaagtccttctcttcgatgagctttttcactttttccacatccagctcttctatcctgtagttgaggtcccccagccacaagatcacatcatggttgctgatggtgagagggggaaggcttgggtcaggctgacaaaactgcattcgagaacaaatgtccttatagtcctggttcctcctctcatactcttcaatgtgggctgccaagtgagaattcacaacgcagatgctggtgttgtggaactggaacctgatcgccacgcctcccttgttgcccatcctccccatgattcctgtccccacagtctcggcttccacttctgagatataagctgcatgctcctgtttgacatataacagcagcataatcccaaccagtcggataagcttcacctttgcatatttggcatctggatgaagaccctctgacacagctttgaaccactcttcctcctttggggtatcgtgaaagaaaaaagcttccttactcagatcaagctcctggaaccctacacaatagacatctggggcctggataccattgctcagccacagccggaggcattctttgggggactgcccatttacattgtatgttcccgcaaaaaacctgaagttctggatataggtgtaatcctcttctttctgtagtagatgtgatttcacaattgtatctcgcagtccaaacttctgcatggataaaatatgagccttgtccgacactgtgatagtggaggagcgaaccatgtcagtaatttcggacttggatttattctgtcttggttgcaagctttctggtttatcttgacccctggagctttggtccataggcactcccttcccatttggtctcaaaccatcaaagttagaaccacctccgccaattgtcgcgtaccctggccaggtaactagggccgagttacaaccgcgcggcgttggcatctccagctccagctctgcgcacctataccgagacagccacaggaattcaggatcccgggtcgcagaatcgaagcctggacaggccctggcaacttcgtggaggaacatcctggtttgtgaaccaaagggcagttggaatacgaggctaagctctgctgtgtccagctggacggtcacatctgagccttgtccataaaatggagatgcaaacagtgataacctcatagagctgtgagaaaagcctgatttaggcccggtgcggtggctcatgcctgtaatcccagcactttgggaggccgaggtggggtggatcacaaggtcaggagatcgagaccatcctggccaacacggtgaaaccccgtctctacaaggatgtagagttcaccatctggggacacttcttccagcgtaaaatcccgcgagactggcactatctggtccagagagacatcgtccccggtaatggccatcctccggtgcgtatagaggaagagagcgtgttcctggccgccgtgctccaggcggtagcgcacgagtcccaggaggcggctctgccggctgtccccctcacacagcacaccttgcaccgcgatgacgcagtattccccctcagccagcgtctcctggattgccacagactggtccatgctggcccctgctgagcgcacacaccctcctgagctgtcaccacagggcgcacgggactccgctgccccaggttccgggacagtgactacattt

SEQ ID NO: 18329 - RNA, 2986 nt, Homo sapiens
  source 1..2986: mol_type = other RNA
tgaagtaccagctactcgagaggctgaggcaggagaattgcttgaaccaaggaggcagaggttgcagtgagccaagaccacgccaacgcactccagcctgggcaacaagagtgaaactccatctcaaaaaagaaaaaaaaaaaaaaaaggccgggcgtggtggctcacatctgtaatcctagcacttggggaggccgaggcaggcagattacctgagttcaggagttttagaacagcctgggcaacacggtgaaaccccgtctctactaaaatgcaaaaaattagctgggcgtggcagtgtgtgcctgcagtcccagctactcgggaggctgaggcaggataattgcttgcacccaggaggcagaggttgcagtgagccgagatcgtgccaccgcactccaccctgcgcgacagagcaaaactccgtctcaaaataaaaaaaaataaaaaataaaaaaatctgtgttaaataactaaagttgaaaattgaatgtcagttttattatggtggattttctcccgtgtcttcacgactcacagcgctgagtgtgctaaccaatggtgggcttaattggggtactaggctcaggaaatagctgccattcttgctaccaagtggcctcacataattatcttaaggcatctcttgagctgaaacaggtggggctggtaattggcagcctcaagtaaaataggaggagagagaggctcagagtgggttgcagaggaactggtgaataaattcttgagccttcttcttctctgtcatatcaagcttttggtgaccagctgggtttcgaagcaataagctgccaaatatgctagctagaatattctcatccaaatgattttttgctgaatttttcagcagttctcgcaaaaacgccatcaagtagtggaagacatttttgtggaatatggggagagtagaaatgacctgtttgcttgctgtgtagttgccagaacactccaagcagttatggtaggtgctgtaacagatgacaggctctggaaggctctccaggaaaagcagcagggcttcggctacagaatgattgctggcagagaggttatcaatcattccagtatccaagcagtccctgatatgttcaaattctgacctcaggcctggttgctgaaacagatcttcctgctggacagcatttcggtacaggtaatcaaccatcatccagagctctttggggatttccatggggctatccaactggctcccatcatctccagtccatactggcatcagagtcagctcactaatggtttcaagtggtaggtccaagattggctctctcatgtaacacagtgtatgaatgggagacccaaaacagctgggcaggtagttcccagacacagacaaaaagtaatcctttcccctgtccaagtgcagaaccagaatgtcctcaattttgtcttcacccgagttgagctttgtagctgtcatcttatttacgaagagctccaagtcaatctcaacatcagaatctggcaggaggaagcctctgctggggttggcattcagccactgcttacagtaagactcttcatcaggcttgttgatgaattcaaaatgacagggtacttgtccattatgaattgtaaaggattctactttcaattgcatgtacttcacattctgaaaacagaactctcgcttggacagggacacagaaggaatgttggcattttccatcttatccagggagcgaacaatttcctccagtgtcttccggtaaagctcgtcatttacgaccctcaccccgatgtcaaacactgagctgacaggcttgtggtcactggtcttcagggccatgtggctctggtaactcagctgagtgatgttcttccctttccagagaatccgatcacaccaggcaggagcacggcacttctcactggtatcccagtcgtcagagcccgtatcatacttgtaagtaggctggaatgtgagctcaccctctgtgaagccttcaaagacagtctttgcggccacctgaattttcagctgatcatatgcatacagcatttgaaagtccttctcttcgatgagctttttcactttttccacatccagctcttctatcctgtagttgaggtcccccagccacaagatcacatcatggttgctgatggtgagagggggaaggcttgggtcaggctgacaaaactgcattcgagaacaaatgtccttatagtcctggttcctcctctcatactcttcaatgtgggctgccaagtgagaattcacaacgcagatgctggtgttgtggaactggaacctgatcgccacgcctcccttgttgcccatcctccccatgattcctgtccccacagtctcggcttccacttctgagatataagctgcatgctcctgtttgacatataacagcagcataatcccaaccagtcggataagcttcacctttgcatatttggcatctggatgaagaccctctgacacagctttgaaccactcttcctcctttggggtatcgtgaaagaaaaaagcttccttactcagatcaagctcctggaaccctacacaatagacatctggggcctggataccattgctcagccacagccggaggcattctttgggggactgcccatttacattgtatgttcccgcaaaaaacctgaagttctggatataggtgtaatcctcttctttctgtagtagatgtgatttcacaattgtatctcgcagtccaaacttctgcatggataaaatatgagccttgtccgacactgtgatagtggaggagcgaaccatgtcagtaatttcggacttggatttattctgtcttggttgcaagctttctggtttatcttgacccctggagctttggtccataggcactcccttcccatttggtctcaaaccatcaaagttagaaccacctgcagtgttgcgctcccgagagccggcggcggcagacatttccctgcctgcttcctcaagctcctc

SEQ ID NO: 18330 - RNA, 2984 nt, Homo sapiens
  source 1..2984: mol_type = other RNA
tgaagtaccagctactcgagaggctgaggcaggagaattgcttgaaccaaggaggcagaggttgcagtgagccaagaccacgccaacgcactccagcctgggcaacaagagtgaaactccatctcaaaaaagaaaaaaaaaaaaaaaaggccgggcgtggtggctcacatctgtaatcctagcacttggggaggccgaggcaggcagattacctgagttcaggagttttagaacagcctgggcaacacggtgaaaccccgtctctactaaaatgcaaaaaattagctgggcgtggcagtgtgtgcctgcagtcccagctactcgggaggctgaggcaggataattgcttgcacccaggaggcagaggttgcagtgagccgagatcgtgccaccgcactccaccctgcgcgacagagcaaaactccgtctcaaaataaaaaaaaataaaaaataaaaaaatctgtgttaaataactaaagttgaaaattgaatgtcagttttattatggtggattttctcccgtgtcttcacgactcacagcgctgagtgtgctaaccaatggtgggcttaattggggtactaggctcaggaaatagctgccattcttgctaccaagtggcctcacataattatcttaaggcatctcttgagctgaaacaggtggggctggtaattggcagcctcaagtaaaataggaggagagagaggctcagagtgggttgcagaggaactggtgaataaattcttgagccttcttcttctctgtcatatcaagcttttggtgaccagctgggtttcgaagcaataagctgccaaatatgctagctagaatattctcatccaaatgattttttgctgaatttttcagcagttctcgcaaaaacgccatcaagtagtggaagacatttttgtggaatatggggagagtagaaatgacctgtttgcttgctgtgtagttgccagaacactccaagcagttatggtaggtgctgtaacagatgacaggctctggaaggctctccaggaaaagcagcagggcttcggctacagaatgattgctggcagagaggttatcaatcattccagtatccaagcagtccctgatatgttcaaattctgacctcaggcctggttgctgaaacagatcttcctgctggacagcatttcggtacaggtaatcaaccatcatccagagctctttggggatttccatggggctatccaactggctcccatcatctccagtccatactggcatcagagtcagctcactaatggtttcaagtggtaggtccaagattggctctctcatgtaacacagtgtatgaatgggagacccaaaacagctgggcaggtagttcccagacacagacaaaaagtaatcctttcccctgtccaagtgcagaaccagaatgtcctcaattttgtcttcacccgagttgagctttgtagctgtcatcttatttacgaagagctccaagtcaatctcaacatcagaatctggcaggaggaagcctctgctggggttggcattcagccactgcttacagtaagactcttcatcaggcttgttgatgaattcaaaatgacagggtacttgtccattatgaattgtaaaggattctactttcaattgcatgtacttcacattctgaaaacagaactctcgcttggacagggacacagaaggaatgttggcattttccatcttatccagggagcgaacaatttcctccagtgtcttccggtaaagctcgtcatttacgaccctcaccccgatgtcaaacactgagctgacaggcttgtggtcactggtcttcagggccatgtggctctggtaactcagctgagtgatgttcttccctttccagagaatccgatcacaccaggcaggagcacggcacttctcactggtatcccagtcgtcagagcccgtatcatacttgtaagtaggctggaatgtgagctcaccctctgtgaagccttcaaagacagtctttgcggccacctgaattttcagctgatcatatgcatacagcatttgaaagtccttctcttcgatgagctttttcactttttccacatccagctcttctatcctgtagttgaggtcccccagccacaagatcacatcatggttgctgatggtgagagggggaaggcttgggtcaggctgacaaaactgcattcgagaacaaatgtccttatagtcctggttcctcctctcatactcttcaatgtgggctgccaagtgagaattcacaacgcagatgctggtgttgtggaactggaacctgatcgccacgcctcccttgttgcccatcctccccatgattcctgtccccacagtctcggcttccacttctgagatataagctgcatgctcctgtttgacatataacagcagcataatcccaaccagtcggataagcttcacctttgcatatttggcatctggatgaagaccctctgacacagctttgaaccactcttcctcctttggggtatcgtgaaagaaaaaagcttccttactcagatcaagctcctggaaccctacacaatagacatctggggcctggataccattgctcagccacagccggaggcattctttgggggactgcccatttacattgtatgttcccgcaaaaaacctgaagttctggatataggtgtaatcctcttctttctgtagtagatgtgatttcacaattgtatctcgcagtccaaacttctgcatggataaaatatgagccttgtccgacactgtgatagtggaggagcgaaccatgtcagtaatttcggacttggatttattctgtcttggttgcaagctttctggtttatcttgacccctggagctttggtccataggcactcccttcccatttggtctcaaaccatcaaagttagaaccacctgcctccgccaattgtcgcgtaccctggccaggtaactagggccgagttacaaccgcgcggcgt

SEQ ID NO: 18331 - RNA, 2982 nt, Homo sapiens
  source 1..2982: mol_type = other RNA
tgaagtaccagctactcgagaggctgaggcaggagaattgcttgaaccaaggaggcagaggttgcagtgagccaagaccacgccaacgcactccagcctgggcaacaagagtgaaactccatctcaaaaaagaaaaaaaaaaaaaaaaggccgggcgtggtggctcacatctgtaatcctagcacttggggaggccgaggcaggcagattacctgagttcaggagttttagaacagcctgggcaacacggtgaaaccccgtctctactaaaatgcaaaaaattagctgggcgtggcagtgtgtgcctgcagtcccagctactcgggaggctgaggcaggataattgcttgcacccaggaggcagaggttgcagtgagccgagatcgtgccaccgcactccaccctgcgcgacagagcaaaactccgtctcaaaataaaaaaaaataaaaaataaaaaaatctgtgttaaataactaaagttgaaaattgaatgtcagttttattatggtggattttctcccgtgtcttcacgactcacagcgctgagtgtgctaaccaatggtgggcttaattggggtactaggctcaggaaatagctgccattcttgctaccaagtggcctcacataattatcttaaggcatctcttgagctgaaacaggtggggctggtaattggcagcctcaagtaaaataggaggagagagaggctcagagtgggttgcagaggaactggtgaataaattcttgagccttcttcttctctgtcatatcaagcttttggtgaccagctgggtttcgaagcaataagctgccaaatatgctagctagaatattctcatccaaatgattttttgctgaatttttcagcagttctcgcaaaaacgccatcaagtagtggaagacatttttgtggaatatggggagagtagaaatgacctgtttgcttgctgtgtagttgccagaacactccaagcagttatggtaggtgctgtaacagatgacaggctctggaaggctctccaggaaaagcagcagggcttcggctacagaatgattgctggcagagaggttatcaatcattccagtatccaagcagtccctgatatgttcaaattctgacctcaggcctggttgctgaaacagatcttcctgctggacagcatttcggtacaggtaatcaaccatcatccagagctctttggggatttccatggggctatccaactggctcccatcatctccagtccatactggcatcagagtcagctcactaatggtttcaagtggtaggtccaagattggctctctcatgtaacacagtgtatgaatgggagacccaaaacagctgggcaggtagttcccagacacagacaaaaagtaatcctttcccctgtccaagtgcagaaccagaatgtcctcaattttgtcttcacccgagttgagctttgtagctgtcatcttatttacgaagagctccaagtcaatctcaacatcagaatctggcaggaggaagcctctgctggggttggcattcagccactgcttacagtaagactcttcatcaggcttgttgatgaattcaaaatgacagggtacttgtccattatgaattgtaaaggattctactttcaattgcatgtacttcacattctgaaaacagaactctcgcttggacagggacacagaaggaatgttggcattttccatcttatccagggagcgaacaatttcctccagtgtcttccggtaaagctcgtcatttacgaccctcaccccgatgtcaaacactgagctgacaggcttgtggtcactggtcttcagggccatgtggctctggtaactcagctgagtgatgttcttccctttccagagaatccgatcacaccaggcaggagcacggcacttctcactggtatcccagtcgtcagagcccgtatcatacttgtaagtaggctggaatgtgagctcaccctctgtgaagccttcaaagacagtctttgcggccacctgaattttcagctgatcatatgcatacagcatttgaaagtccttctcttcgatgagctttttcactttttccacatccagctcttctatcctgtagttgaggtcccccagccacaagatcacatcatggttgctgatggtgagagggggaaggcttgggtcaggctgacaaaactgcattcgagaacaaatgtccttatagtcctggttcctcctctcatactcttcaatgtgggctgccaagtgagaattcacaacgcagatgctggtgttgtggaactggaacctgatcgccacgcctcccttgttgcccatcctccccatgattcctgtccccacagtctcggcttccacttctgagatataagctgcatgctcctgtttgacatataacagcagcataatcccaaccagtcggataagcttcacctttgcatatttggcatctggatgaagaccctctgacacagctttgaaccactcttcctcctttggggtatcgtgaaagaaaaaagcttccttactcagatcaagctcctggaaccctacacaatagacatctggggcctggataccattgctcagccacagccggaggcattctttgggggactgcccatttacattgtatgttcccgcaaaaaacctgaagttctggatataggtgtaatcctcttctttctgtagtagatgtgatttcacaattgtatctcgcagtccaaacttctgcatggataaaatatgagccttgtccgacactgtgatagtggaggagcgaaccatgtcagtaatttcggacttggatttattcttggttgcaagctttctggtttatcttgacccctggagctttggtccataggcactcccttcccatttggtctcaaaccatcaaagttagaaccacctgcagtgttgcgctcccgagagccggcggcggcagacatttccctgcctgcttcctcaagctcctc

SEQ ID NO: 18332 - RNA, 1164 nt, Homo sapiens
  source 1..1164: mol_type = other RNA
tgaagtaccagctactcgagaggctgaggcaggagaattgcttgaacccgggaagcgggggttgccgtgagccgagatcgtgccattgcattccagcctgggcaacaagagtgaaactccgtctcaaaaaaaaaaaaaaaaaaaaaaaagagattctcctacctcagcttcccgagtagctgggattacaggcatgcaccaccacaatgcccggctaattttgtatttttagtagagacggggtttctccatggtggtcaggctggtctcgaactcctgacttcaggtgatccacccatcttggcctcccaaagtgctgggattacaggcatgagccaccgcgcctggctgacttcctcttttattacttatcttcttgaccctgccttggctgttgggctctaagagcatacaaattctaccacctccagctaccaatgcgagccaagttctgagccttgagtgggaatgtggcacaactgggcactgggtaattaagtcctgggtccaggccaaaggaggacccagccttatatggagttcataggacagaggcacatgactttcttaggaggcagccaaaggcctctggactgatcagggcatcggtggcagaggagcagggtgacaggccgcctttggctgggctttatctgggctgatgctgaagctgtagaggccctggagcacaccattcaccaccacgttgggcagcgactctggggaggggttgcaaacatagggatccacatggaagctcaggacaggccgctggtgctgctgggagctgctgtcgccaggcaggaactccctcagggtgccccagttgctagccttggggtctgtggggaagtgccgaagtctcaggaattccagtaactccttgggcacctcctggttcaggtacaggatgccctggatgtaagcctccaagccctgccggcgctgttccaaccctctggtcctccagttgggcaggcgtttcgaggggaagtcgggcactttgtacagcttcttgatcatgtggcttttctccgggctctgcctgggcccctcggcctcgggccccaccgacgggatgtgaacttccagcatccgcgccccggccccagctgctccgcgcgctcggctcggagccctaactctcccggagcggactgagga

SEQ ID NO: 18333 - RNA, 1224 nt, Homo sapiens
  source 1..1224: mol_type = other RNA
tgaagtaccagctactcgagaggctgaggcaggagaattgcttgaacccgggaagcgggggttgccgtgagccgagatcgtgccattgcattccagcctgggcaacaagagtgaaactccgtctcaaaaaaaaaaaaaaaaaaaaaaaagagattctcctacctcagcttcccgagtagctgggattacaggcatgcaccaccacaatgcccggctaattttgtatttttagtagagacggggtttctccatggtggtcaggctggtctcgaactcctgacttcaggtgatccacccatcttggcctcccaaagtgctgggattacaggcatgagccaccgcgcctggctgacttcctcttttattacttatcttcttgaccctgccttggctgttgggctctaagagcatacaaattctaccacctccagctaccaatgcgagccaagttctgagccttgagtgggaatgtggcacaactgggcactgggtaattaagtcctgggtccaggccaaaggaggacccagccttatatggagttcataggacagaggcacatgactttcttaggaggcagccaaaggcctctggactgatcagggcatcggtggcagaggagcagggtgacaggccgcctttggctgggctttatctgggctgatgctgaagctgtagaggccctggagcacaccattcaccaccacgttgggcagcgactctggggaggggttgcaaacatagggatccacatggaagctcaggacaggccgctggtgctgctgggagctgctgtcgccaggcaggaactccctcagggtgccccagttgctagccttggggtctgtggggaagtgccgaagtctcaggaattccagtaactccttgggcacctcctggttcaggtacaggatgccctggatgtaagcctccaagccctgccggcgctgttccaaccctctggtcctccagttgggcaggcgtttcgaggggaagtcgggcactttgtacagcttcttgatccgcttgtgcagcgcgtggaactcgctgtagcgccttggcaccgtgtgtctgcgcccgctgcacagcacctccactcggaacaccatgtggcttttctccgggctctgcctgggcccctcggcctcgggccccaccgacgggatgtgaacttccagcatccgcgccccggccccagctgctccgcgcgctcggctcggagccct

SEQ ID NO: 18334 - RNA, 1271 nt, Homo sapiens
  source 1..1271: mol_type = other RNA
tgaagtaccagctactcgagaggctgaggcaggagaattgcttgaacccgggaagcgggggttgccgtgagccgagatcgtgccattgcattccagcctgggcaacaagagtgaaactccgtctcaaaaaaaaaaaaaaaaaaaaaaaagagattctcctacctcagcttcccgagtagctgggattacaggcatgcaccaccacaatgcccggctaattttgtatttttagtagagacggggtttctccatggtggtcaggctggtctcgaactcctgacttcaggtgatccacccatcttggcctcccaaagtgctgggattacaggcatgagccaccgcgcctggctgacttcctcttttattacttatcttcttgaccctgccttggctgttgggctctaagagcatacaaattctaccacctccagctaccaatgcgagccaagttctgagccttgagtgggaatgtggcacaactgggcactgggtaattaagtcctgggtccaggccaaaggaggacccagccttatatggagttcataggacagaggcacatgactttcttaggaggcagccaaaggcctctggactgatcagggcatcggtggcagaggagcagggtgacaggccgcctttggctgggctttatctgggctgatgctgaagctgtagaggccctggagcacaccattcaccaccacgttgggcagcgactctggggaggggttgcaaacatagggatccacatggaagctcaggacaggccgctggtgctgctgggagctgctgtcgccaggcaggaactccctcagggtgctgctcactgctgacagcccctggcccccgccatcggccccccttacccccagttgctagccttggggtctgtggggaagtgccgaagtctcaggaattccagtaactccttgggcacctcctggttcaggtacaggatgccctggatgtaagcctccaagccctgccggcgctgttccaaccctctggtcctccagttgggcaggcgtttcgaggggaagtcgggcactttgtacagcttcttgatccgcttgtgcagcgcgtggaactcgctgtagcgccttggcaccgtgtgtctgcgcccgctgcacagcacctccactcggaacaccatgtggcttttctccgggctctgcctgggcccctcggcctcgggccccaccgacgggatgtgaacttccagcatccgcgccccggccccagctgctccgcgcgctcggctcggagccct

SEQ ID NO: 18335 - RNA, 1108 nt, Homo sapiens
  source 1..1108: mol_type = other RNA
tgaagtaccagctactcgagaggctgaggcaggagaattgcttgaaccctggaggtagaggttgcagtgagccgagatcgtgccactgctctccagcctgagcaacagagtgagactccattgtggatcaggtaccatgctagtgcctcactctttaggaacactagatataatgatctcgaacccgggcaagcctcacaaccttctttagcttctcattccggaagatttctctgctgaaggtatccagccgggggttggcaactctggccacctttttaccttggacttcctgcacctcaataacaccaggtgagaagcacctgctcaactcctcagctgcctccccttccacgggctcaagcagggtgatgtctggcaggagcctgtaactggctgttgccactggtgaaaacttggcatgatctttgccaatgcccttgacacagtgcatgagcaggtcaatttcttggccaggccgcagctgagcgatgaggatatcatcatgcactggtcggatagtgccctctggaaagagatcagcctggttccccagggggatccatgtcatatgcctggtatacactttgtggttcacgtacagttcgttggggtcagaggaatctttagcagcatgggggttccgagtgcatctgacctggagacgaaactgtagagtatctatctctgtgccttcttcatctccttggttccgatactcaaaaagacggggatcagcatgaatgggaatgagccccagacggtgagcaagaatctcatcctgaacaatggatgtattattgtacaccaggaccttctccacagccatagttggcacctcagctagcagaattcgtcgaaaagcattggcaatggctgcgtcaattcccaccatgtcaaactccagtgagttttcatccatgtgtactacatccacacggaaattcttctcgaagcggtcctggtcccaggcatcatcataaccggaatagttaccgggaaagtcagtagtatggacattgcgaaccccaaactcccccagaaccacgcggctccgcatttcctccaccgcctgagaagccgccatcttcaatctctccacgagact

SEQ ID NO: 18336 - RNA, 6007 nt, Homo sapiens
  source 1..6007: mol_type = other RNA
tgaagtaccagctactcgagaggctgaggcaggcaaattgcttcaaacctgtgaggcagaggttgcagtgagccgggatcgcaccactgcactccaggctgggctacagggtgagattctgtctccaaaaaaaaaaaaaagagagaaaggaatagagtgttttgttagctctggtcattcccactcttcttctctcttgttgctattactttgaagcatttggtttggttattctattttgttaaggaataattaaaaagtacattactaacagttttgctttatatattgtgtgccttgggcaaaatttgtgtgtgtggttattcacagaggaggagccagataggtagctcagtccataaactatggaaggtagcagtatcctttactgcagtggctttcaaatttgacatgcaccaaaatctcctggagagcttgttaaaacatagaaagcagggcctcatcccccacgtttttgattcagtaggtctgggttggggctcgagaatttgcatttctaacaaattcctaggtgatgctgatgctgatgctgatgcttctggtttggagcacatactttgagaaccactgctctaatggaatcagtagtcacaaggccaagcagccaggtagacactaagggaaaacagtacctccctgtgtaggttttcaggacacaacattagttacaagttttatcacctgctcaaccaggtatatagctatgtcaattctcaagggctttaactgacaaaaccagttgttagaggacagttctttcaagggtgaacccaacacctaaaaaaagttttgaaaaagtcagttatttgcctatttaaggacggttttagaatccactattatgggaatggatctgcttagcctatttgaggtttttttgttttttgagacagagtctcgccctgttgcctgggctggagtgcaatggtgcgattttgactcactgaaacctctgcctcccgggttcaagtgattcgcctccctcagcctcccgagtagctgggattacaggcgcccgccaccacgcctggctatttttttttgtatttttagtagagatggggtttcaccatgttggccaggttggtctcaaactcttggcctcgtgattcgcccaccttggcctcccaaagtgctgggattacaggtgtaagtcactgtgcctggccgcctagtggagttttaatgccaatatccttggactaacttgaaaatgaataatataaattcgaaatttctgcctgcagtacaattcaaaataagagtttctaaatttttttaatccttatgttaaaataataaataatctcatttcagttgttttttcacccaattactaaaaaacaaaatagtcataaaaaagaattcatttagcaaaggtactatttgtagatattagccacttattaaaaacatatttctattaagattgttcttacattcttagatttagaacacctgatatctggacccagctgagtttttattttacagatcataaaacggatgaaagtatatcacagtaattaatgaagccgttctaatttagcttgaagagatttaaaattcccagtgatggcttgtactgctactgacgagctcatagactggagctcaacaaggtaaccacaaacagcatccaggcagagatttgtaaatcttctcctttcacaatttaaaacttggctgggattctcaacatatcttatcaataatacatgtatacaatccaaaaggtgcagtggcttcttcattctgttccagaatggatcccgtgatttgaacaactgatcataaacttctagtagtctaggtaatggtactccaatttcattcattgtctgtattacgaagcccacatcccagttcaaagtacaaacctgctgttctaaaaactgtacaataaaatctaaaggaaagaagcgtggtgtgccagcataaattttgccaaggagaacaatcttgagactaagagcatgcattctatccgaggagctcaatgtcacactgtcactcaattctttctctatgatatcttgccaaagtgtctgcaccaatatagggtctgaataaccggcacaatgaattattgcaagtttgcactctgcaagtttaaatgggtcagcaaattccccataaagcttagttatgtccatcagctcagaatccagctgagaaactgcatcctgtacagaagaatgatgggaatactgcctttgtagtgtctcctgtatctgaagttggatcctagcaacctccattttttcttctaattcatgaagaaattcaccatcggcagctattgatgaaatggcagtggaacttttggcactaagaatggctcgagcaatgtactctagtcgctgctgaagtgaaatttctgtgctatgcatgtcagccagtctggacagtacacgagcagcattactgaaacttctgttcttctcgtaataccgccagagtaaatccatataacgaactctgttttgatcaactttggccattcggactagatgtggctccagaaatggagaagcaacctgtagcagcttatctgcaaggtcgacttgtattagccaattataaagggcaatactaaagagctcatccttggatcgctgtgacaatttaagcatttgttcaaaatgatgtcctgcttcttcattactcagcatatttggatcagatgacaacactggaggaccaggttttttgggtacactgggagactgaggagcggccttactttgatttaccagttcttgaagtgtgtctgtaatgcatttgtaactgtttaatctttcttggaaggcctgaagtccaactatgtcttcttctggttctccatgtttatagaaatgaagcccaagaccttgaggatcttttttctctgcagccgtaagagaaagttccaccacaccctcataaaatctcacttgtctatactgagcacaaacattggaaaggtccacttgattgctaattttttgatattcctttaatgattcccttaacattctttctttttcagtcttattttgaacttgtcgggaacgctggagaagctcatttgccttagaacaaattgcatcatcagtgctatatagaagtgggcagatatcctgtaaatgtaaactaatgccatcaacagcggcattatctctgatgtagcagttgataagagaagcaattaatgcccctgtgagttctttgtccctgattacaagatctttaaaggtggtgatcttcagctgctcttgaagttccttctgaagttctgccacaatgatagtgaattgatgttcacaaagaagtttccataaagccagagcctgatatgattttcgaaccaactgctgaattgcctgaagtgaaatcttttcacttagttgagcctcatgaaacttcctctgcagttcctgttgcatttgctggggatttccgttttcaggacgcatgaatcctatcagcctctgctgcactttagcagtagtatttggatttcctaatggtcctcctgcaaactgggagtttctgtctagaaattcctgcaaaccctttagttcttgtagcactgactctagcagttggcagggaacactactttcaattgcagtgatctctctgttgccactcttgaatattctctccacaactaagcttgcatcccaaatgtttcccatgatccgagaaaagtaaatgcaaataccattgtgttttccagagtacacaatctctggtccagtcacacaactcatatttgtggcctgagttgctgggtttcccagagcacacactggagttgacatggcaggaggctgtataccatgagacggtgttcccaaaaaggatggatttggatagggactaccactaggaacaggagaactagaatagacaggagaccccaagatgggaccaacattacttggaggcggaagagtggttggaaatctcatctgtgcttcaccaccatacctaaagaaagcccgagtagcccaggcagatacttctctatcacaggcagcagtggagcaagcaagaataaggcaagttgcacaagcctggtcttcctgatgtaatttaaagaatctttcaatctcttctccatctcctcccacattactcacaagtagatgcctcagttgatctacaggtctaagtttatgaaacataaggctcccctgtgctgagaggagaacaaatttcttcggaggtaacatgtgctgctgtacaacaactggtgaatcagttattggaatatgatccttgtttaaaggtgtaattattttatctactttcaattcatctatcgcagaaagagcccaggaatgaccatcaacaccagctgtcatctgggtttccatcattggcttttggaaaggaaaagtatcatggttgacacaccataaaatatcattatcctcattttctgaggctgccatcaatagaatacctttactataaagagctctatgtacttttgaaggcttttccacggttgaagatgctgagaatccaggaggtaagcggacatgaaccagcgtcagtgtattaggccgtgctaatggctgtctgaatggacaagtgctaaaatataacctaacacctgcatgtgtgacagccaataactgacagtccagtgattcagaattttcaatcactgctatttggacaattggtttaaaaacagaacgatcgatggtcctagcaatgttaccagcagcagagacaatggcattctgtgacacagaggcaactctgctcattccttgtccatcttgtcccaaatcatacacctgtattactcctttctcagatcgtgtatataaaatatttctagaattatcaattgcaatttgaagaataggatcatcttctgagaacgtgaattgtagcaaggaaggaacaaggaaagaaagtgagctctttgagtggtttattttcctacatctttggctaaaccaccctgcttcagcctggtaggctacttcatataaacagccatcctttccagccaagaaaattctgccattatcagtggaagttattgttaaaaggtaagtattatcagtaggaagagaatataaaggatctggaagcaactgcattccaccagacaaactatcattaagaactccagaacctgtttgcaaattagcatagctgagtccaagaattactatgtctacaggggtcgccaaaaccaggaggtgtcgcacatgaggttgaaagatgcctgcttttggcttcacaagccccacagcaagaatagtctcactaagtccatcaaaataggcaaggtctcctccatcctcatagttccacatgaatatatcactgtcaattgtgagccaagctctgctgataggagggaacacacccatcatgcaattacactgcatatgtccaaactgctcaacaagttcaggtgggagaggaactcttcggatggaactgatctctggaaggttgggtacggacagcaaaccaggtccttgcaaaggataatccatatctgacatgccagaaacggtgggattatctgaaaagaagctgcttgctgttctccaaaaatgcagccaacagtgccataaatctcagcatatcctcgccgggaccaacgctggggataagtagcaaattaggaagtcaggcgagagtcctttaggttgagaaagcagggtcactatcactcacttggggcagacaccataagcagctcggaaaggtccgggtacatgcggtcctcttgcaactgacggtcgatgagccgtccagcattttccagagcttcctgcagggctgcggcagatgtagaggccggcatcgccgcgcccaacaaagaagacggcatctcggaaatcgtagacaccagggtccagaaaaagtcaaaaaccaaggagaaacaagaaaagatccaagaagttagcttagatccgccgcctagggcgcgcgcgccaaacgagcgccttggcgcctcgac

SEQ ID NO: 18337 - RNA, 5852 nt, Homo sapiens
  source 1..5852: mol_type = other RNA
tgaagtaccagctactcgagaggctgaggcaggcaaattgcttcaaacctgtgaggcagaggttgcagtgagccgggatcgcaccactgcactccaggctgggctacagggtgagattctgtctccaaaaaaaaaaaaaagagagaaaggaatagagtgttttgttagctctggtcattcccactcttcttctctcttgttgctattactttgaagcatttggtttggttattctattttgttaaggaataattaaaaagtacattactaacagttttgctttatatattgtgtgccttgggcaaaatttgtgtgtgtggttattcacagaggaggagccagataggtagctcagtccataaactatggaaggtagcagtatcctttactgcagtggctttcaaatttgacatgcaccaaaatctcctggagagcttgttaaaacatagaaagcagggcctcatcccccacgtttttgattcagtaggtctgggttggggctcgagaatttgcatttctaacaaattcctaggtgatgctgatgctgatgctgatgcttctggtttggagcacatactttgagaaccactgctctaatggaatcagtagtcacaaggccaagcagccaggtagacactaagggaaaacagtacctccctgtgtaggttttcaggacacaacattagttacaagttttatcacctgctcaaccaggtatatagctatgtcaattctcaagggctttaactgacaaaaccagttgttagaggacagttctttcaagggtgaacccaacacctaaaaaaagttttgaaaaagtcagttatttgcctatttaaggacggttttagaatccactattatgggaatggatctgcttagcctatttgaggtttttttgttttttgagacagagtctcgccctgttgcctgggctggagtgcaatggtgcgattttgactcactgaaacctctgcctcccgggttcaagtgattcgcctccctcagcctcccgagtagctgggattacaggcgcccgccaccacgcctggctatttttttttgtatttttagtagagatggggtttcaccatgttggccaggttggtctcaaactcttggcctcgtgattcgcccaccttggcctcccaaagtgctgggattacaggtgtaagtcactgtgcctggccgcctagtggagttttaatgccaatatccttggactaacttgaaaatgaataatataaattcgaaatttctgcctgcagtacaattcaaaataagagtttctaaatttttttaatccttatgttaaaataataaataatctcatttcagttgttttttcacccaattactaaaaaacaaaatagtcataaaaaagaattcatttagcaaaggtactatttgtagatattagccacttattaaaaacatatttctattaagattgttcttacattcttagatttagaacacctgatatctggacccagctgagtttttattttacagatcataaaacggatgaaagtatatcacagtaattaatgaagccgttctaatttagcttgaagagatttaaaattcccagtgatggcttgtactgctactgacgagctcatagactggagctcaacaaggtaaccacaaacagcatccaggcagagatttgtaaatcttctcctttcacaatttaaaacttggctgggattctcaacatatcttatcaataatacatgtatacaatccaaaaggtgcagtggcttcttcattctgttccagaatggatcccgtgatttgaacaactgatcataaacttctagtagtctaggtaatggtactccaatttcattcattgtctgtattacgaagcccacatcccagttcaaagtacaaacctgctgttctaaaaactgtacaataaaatctaaaggaaagaagcgtggtgtgccagcataaattttgccaaggagaacaatcttgagactaagagcatgcattctatccgaggagctcaatgtcacactgtcactcaattctttctctatgatatcttgccaaagtgtctgcaccaatatagggtctgaataaccggcacaatgaattattgcaagtttgcactctgcaagtttaaatgggtcagcaaattccccataaagcttagttatgtccatcagctcagaatccagctgagaaactgcatcctgtacagaagaatgatgggaatactgcctttgtagtgtctcctgtatctgaagttggatcctagcaacctccattttttcttctaattcatgaagaaattcaccatcggcagctattgatgaaatggcagtggaacttttggcactaagaatggctcgagcaatgtactctagtcgctgctgaagtgaaatttctgtgctatgcatgtcagccagtctggacagtacacgagcagcattactgaaacttctgttcttctcgtaataccgccagagtaaatccatataacgaactctgttttgatcaactttggccattcggactagatgtggctccagaaatggagaagcaacctgtagcagcttatctgcaaggtcgacttgtattagccaattataaagggcaatactaaagagctcatccttggatcgctgtgacaatttaagcatttgttcaaaatgatgtcctgcttcttcattactcagcatatttggatcagatgacaacactggaggaccaggttttttgggtacactgggagactgaggagcggccttactttgatttaccagttcttgaagtgtgtctgtaatgcatttgtaactgtttaatctttcttggaaggcctgaagtccaactatgtcttcttctggttctccatgtttatagaaatgaagcccaagaccttgaggatcttttttctctgcagccgtaagagaaagttccaccacaccctcataaaatctcacttgtctatactgagcacaaacattggaaaggtccacttgattgctaattttttgatattcctttaatgattcccttaacattctttctttttcagtcttattttgaacttgtcgggaacgctggagaagctcatttgccttagaacaaattgcatcatcagtgctatatagaagtgggcagatatcctgtaaatgtaaactaatgccatcaacagcggcattatctctgatgtagcagttgataagagaagcaattaatgcccctgtgagttctttgtccctgattacaagatctttaaaggtggtgatcttcagctgctcttgaagttccttctgaagttctgccacaatgatagtgaattgatgttcacaaagaagtttccataaagccagagcctgatatgattttcgaaccaactgctgaattgcctgaagtgaaatcttttcacttagttgagcctcatgaaacttcctctgcagttcctgttgcatttgctggggatttccgttttcaggacgcatgaatcctatcagcctctgctgcactttagcagtagtatttggatttcctaatggtcctcctgcaaactgggagtttctgtctagaaattcctgcaaaccctttagttcttgtagcactgactctagcagttggcagggaacactactttcaattgcagtgatctctctgttgccactcttgaatattctctccacaactaagcttgcatcccaaatgtttcccatgatccgagaaaagtaaatgcaaataccattgtgttttccagagtacacaatctctggtccagtcacacaactcatatttgtggcctgagttgctgggtttcccagagcacacactggagttgacatggcaggaggctgtataccatgagacggtgttcccaaaaaggatggatttggatagggactaccactaggaacaggagaactagaatagacaggagaccccaagatgggaccaacattacttggaggcggaagagtggttggaaatctcatctgtgcttcaccaccatacctaaagaaagcccgagtagcccaggcagatacttctctatcacaggcagcagtggagcaagcaagaataaggcaagttgcacaagcctggtcttcctgatgtaatttaaagaatctttcaatctcttctccatctcctcccacattactcacaagtagatgcctcagttgatctacaggtctaagtttatgaaacataaggctcccctgtgctgagaggagaacaaatttcttcggaggtaacatgtgctgctgtacaacaactggtgaatcagttattggaatatgatccttgtttaaaggtgtaattattttatctactttcaattcatctatcgcagaaagagcccaggaatgaccatcaacaccagctgtcatctgggtttccatcattggcttttggaaaggaaaagtatcatggttgacacaccataaaatatcattatcctcattttctgaggctgccatcaatagaatacctttactataaagagctctatgtacttttgaaggcttttccacggttgaagatgctgagaatccaggaggtaagcggacatgaaccagcgtcagtgtattaggccgtgctaatggctgtctgaatggacaagtgctaaaatataacctaacacctgcatgtgtgacagccaataactgacagtccagtgattcagaattttcaatcactgctatttggacaattggtttaaaaacagaacgatcgatggtcctagcaatgttaccagcagcagagacaatggcattctgtgacacagaggcaactctgctcattccttgtccatcttgtcccaaatcatacacctgtattactcctttctcagatcgtgtatataaaatatttctagaattatcaattgcaatttgaagaataggatcatcttctgagaacgtgaattgtagcaaggaaggaacaaggaaagaaagtgagctctttgagtggtttattttcctacatctttggctaaaccaccctgcttcagcctggtaggctacttcatataaacagccatcctttccagccaagaaaattctgccattatcagtggaagttattgttaaaaggtaagtattatcagtaggaagagaatataaaggatctggaagcaactgcattccaccagacaaactatcattaagaactccagaacctgtttgcaaattagcatagctgagtccaagaattactatgtctacaggggtcgccaaaaccaggaggtgtcgcacatgaggttgaaagatgcctgcttttggcttcacaagccccacagcaagaatagtctcactaagtccatcaaaataggcaaggtctcctccatcctcatagttccacatgaatatatcactgtcaattgtgagccaagctctgctgataggagggaacacacccatcatgcaattacactgcatatgtccaaactgctcaacaagttcaggtgggagaggaactcttcggatggaactgatctctggaaggttgggtacggacagcaaaccaggtccttgcaaaggataatccatatctgacatgccagaaacggtgggattatttggggcagacaccataagcagctcggaaaggtccgggtacatgcggtcctcttgcaactgacggtcgatgagccgtccagcattttccagagcttcctgcagggctgcggcagatgtagaggccggcatcgccgcgcccaacaaagaagacggcatctcggaaatcgtagacaccagggtccagaaaaagtcaaaaaccaaggagaaacaagaaaagatccaagaagttagcttagatccgccgcctagggcgcgcgcgccaaacgagcgccttggcgcctcgac

SEQ ID NO: 18338 - RNA, 5660 nt, Homo sapiens
  source 1..5660: mol_type = other RNA
tgaagtaccagctactcgagaggctgaggcaggcaaattgcttcaaacctgtgaggcagaggttgcagtgagccgggatcgcaccactgcactccaggctgggctacagggtgagattctgtctccaaaaaaaaaaaaaagagagaaaggaatagagtgttttgttagctctggtcattcccactcttcttctctcttgttgctattactttgaagcatttggtttggttattctattttgttaaggaataattaaaaagtacattactaacagttttgctttatatattgtgtgccttgggcaaaatttgtgtgtgtggttattcacagaggaggagccagataggtagctcagtccataaactatggaaggtagcagtatcctttactgcagtggctttcaaatttgacatgcaccaaaatctcctggagagcttgttaaaacatagaaagcagggcctcatcccccacgtttttgattcagtaggtctgggttggggctcgagaatttgcatttctaacaaattcctaggtgatgctgatgctgatgctgatgcttctggtttggagcacatactttgagaaccactgctctaatggaatcagtagtcacaaggccaagcagccaggtagacactaagggaaaacagtacctccctgtgtaggttttcaggacacaacattagttacaagttttatcacctgctcaaccaggtatatagctatgtcaattctcaagggctttaactgacaaaaccagttgttagaggacagttctttcaagggtgaacccaacacctaaaaaaagttttgaaaaagtcagttatttgcctatttaaggacggttttagaatccactattatgggaatggatctgcttagcctatttgaggtttttttgttttttgagacagagtctcgccctgttgcctgggctggagtgcaatggtgcgattttgactcactgaaacctctgcctcccgggttcaagtgattcgcctccctcagcctcccgagtagctgggattacaggcgcccgccaccacgcctggctatttttttttgtatttttagtagagatggggtttcaccatgttggccaggttggtctcaaactcttggcctcgtgattcgcccaccttggcctcccaaagtgctgggattacaggtgtaagtcactgtgcctggccgcctagtggagttttaatgccaatatccttggactaacttgaaaatgaataatataaattcgaaatttctgcctgcagtacaattcaaaataagagtttctaaatttttttaatccttatgttaaaataataaataatctcatttcagttgttttttcacccaattactaaaaaacaaaatagtcataaaaaagaattcatttagcaaaggtactatttgtagatattagccacttattaaaaacatatttctattaagattgttcttacattcttagatttagaacacctgatatctggacccagctgagtttttattttacagatcataaaacggatgaaagtatatcacagtaattaatgaagccgttctaatttagcttgaagagatttaaaattcccagtgatggcttgtactgctactgacgagctcatagactggagctcaacaaggtaaccacaaacagcatccaggcagagatttgtaaatcttctcctttcacaatttaaaacttggctgggattctcaacatatcttatcaataatacatgtatacaatccaaaaggtgcagtggcttcttcattctgttccagaatggatcccgtgatttgaacaactgatcataaacttctagtagtctaggtaatggtactccaatttcattcattgtctgtattacgaagcccacatcccagttcaaagtacaaacctgctgttctaaaaactgtacaataaaatctaaaggaaagaagcgtggtgtgccagcataaattttgccaaggagaacaatcttgagactaagagcatgcattctatccgaggagctcaatgtcacactgtcactcaattctttctctatgatatcttgccaaagtgtctgcaccaatatagggtctgaataaccggcacaatgaattattgcaagtttgcactctgcaagtttaaatgggtcagcaaattccccataaagcttagttatgtccatcagctcagaatccagctgagaaactgcatcctgtacagaagaatgatgggaatactgcctttgtagtgtctcctgtatctgaagttggatcctagcaacctccattttttcttctaattcatgaagaaattcaccatcggcagctattgatgaaatggcagtggaacttttggcactaagaatggctcgagcaatgtactctagtcgctgctgaagtgaaatttctgtgctatgcatgtcagccagtctggacagtacacgagcagcattactgaaacttctgttcttctcgtaataccgccagagtaaatccatataacgaactctgttttgatcaactttggccattcggactagatgtggctccagaaatggagaagcaacctgtagcagcttatctgcaaggtcgacttgtattagccaattataaagggcaatactaaagagctcatccttggatcgctgtgacaatttaagcatttgttcaaaatgatgtcctgcttcttcattactcagcatatttggatcagatgacaacactggaggaccaggttttttgggtacactgggagactgaggagcggccttactttgatttaccagttcttgaagtgtgtctgtaatgcatttgtaactgtttaatctttcttggaaggcctgaagtccaactatgtcttcttctggttctccatgtttatagaaatgaagcccaagaccttgaggatcttttttctctgcagccgtaagagaaagttccaccacaccctcataaaatctcacttgtctatactgagcacaaacattggaaaggtccacttgattgctaattttttgatattcctttaatgattcccttaacattctttctttttcagtcttattttgaacttgtcgggaacgctggagaagctcatttgccttctgaagttctgccacaatgatagtgaattgatgttcacaaagaagtttccataaagccagagcctgatatgattttcgaaccaactgctgaattgcctgaagtgaaatcttttcacttagttgagcctcatgaaacttcctctgcagttcctgttgcatttgctggggatttccgttttcaggacgcatgaatcctatcagcctctgctgcactttagcagtagtatttggatttcctaatggtcctcctgcaaactgggagtttctgtctagaaattcctgcaaaccctttagttcttgtagcactgactctagcagttggcagggaacactactttcaattgcagtgatctctctgttgccactcttgaatattctctccacaactaagcttgcatcccaaatgtttcccatgatccgagaaaagtaaatgcaaataccattgtgttttccagagtacacaatctctggtccagtcacacaactcatatttgtggcctgagttgctgggtttcccagagcacacactggagttgacatggcaggaggctgtataccatgagacggtgttcccaaaaaggatggatttggatagggactaccactaggaacaggagaactagaatagacaggagaccccaagatgggaccaacattacttggaggcggaagagtggttggaaatctcatctgtgcttcaccaccatacctaaagaaagcccgagtagcccaggcagatacttctctatcacaggcagcagtggagcaagcaagaataaggcaagttgcacaagcctggtcttcctgatgtaatttaaagaatctttcaatctcttctccatctcctcccacattactcacaagtagatgcctcagttgatctacaggtctaagtttatgaaacataaggctcccctgtgctgagaggagaacaaatttcttcggaggtaacatgtgctgctgtacaacaactggtgaatcagttattggaatatgatccttgtttaaaggtgtaattattttatctactttcaattcatctatcgcagaaagagcccaggaatgaccatcaacaccagctgtcatctgggtttccatcattggcttttggaaaggaaaagtatcatggttgacacaccataaaatatcattatcctcattttctgaggctgccatcaatagaatacctttactataaagagctctatgtacttttgaaggcttttccacggttgaagatgctgagaatccaggaggtaagcggacatgaaccagcgtcagtgtattaggccgtgctaatggctgtctgaatggacaagtgctaaaatataacctaacacctgcatgtgtgacagccaataactgacagtccagtgattcagaattttcaatcactgctatttggacaattggtttaaaaacagaacgatcgatggtcctagcaatgttaccagcagcagagacaatggcattctgtgacacagaggcaactctgctcattccttgtccatcttgtcccaaatcatacacctgtattactcctttctcagatcgtgtatataaaatatttctagaattatcaattgcaatttgaagaataggatcatcttctgagaacgtgaattgtagcaaggaaggaacaaggaaagaaagtgagctctttgagtggtttattttcctacatctttggctaaaccaccctgcttcagcctggtaggctacttcatataaacagccatcctttccagccaagaaaattctgccattatcagtggaagttattgttaaaaggtaagtattatcagtaggaagagaatataaaggatctggaagcaactgcattccaccagacaaactatcattaagaactccagaacctgtttgcaaattagcatagctgagtccaagaattactatgtctacaggggtcgccaaaaccaggaggtgtcgcacatgaggttgaaagatgcctgcttttggcttcacaagccccacagcaagaatagtctcactaagtccatcaaaataggcaaggtctcctccatcctcatagttccacatgaatatatcactgtcaattgtgagccaagctctgctgataggagggaacacacccatcatgcaattacactgcatatgtccaaactgctcaacaagttcaggtgggagaggaactcttcggatggaactgatctctggaaggttgggtacggacagcaaaccaggtccttgcaaaggataatccatatctgacatgccagaaacggtgggattatttggggcagacaccataagcagctcggaaaggtccgggtacatgcggtcctcttgcaactgacggtcgatgagccgtccagcattttccagagcttcctgcagggctgcggcagatgtagaggccggcatcgccgcgcccaacaaagaagacggcatctcggaaatcgtagacaccagggtccagaaaaagtcaaaaaccaaggagaaacaagaaaagatccaagaagttagcttagatccgccgcctagggcgcgcgcgccaaacgagcgccttggcgcctcgac

SEQ ID NO: 18339 - RNA, 8751 nt, Homo sapiens
  source 1..8751: mol_type = other RNA
tgaagtaccagctactcgagaggctgaggcaggggaatcctttgaacccgggaggtggaggttggagtgagccgagatcgcgccactgcactccagcctgacgacagagcaagactccatcaaaacaaaacaaaacaaaacaaaacaaaaaaacaaaacagaacaaaaaccttgagatgaagagattattctggattacacagatgcagctattgtaatcacatgagtccttaaatatgtaagggagaggaagaagaggaagtcagtgatgtcatgtgagaaggtcttgaccaggttgctggatttgaagatggaaggaaactaagcaaaggactctagaagcagggaacagcaagattctctcttggaagcatccaggaaatgcctcctacattctgtagcccaccaagactaagatctttgctgaatgtctgactgacagagctgtaagataataaatttgtgttgttttaggccgttatcgttgtagtaatgtagtaatattttacagcagttctaaaaatctcattttgacaccacattctaaatatggtagacagttaaaaagcctgcgccaaattatttcatctgtaatgctggaaagtctattatttaaatgctgattttcagactttagtactttcacattaaagatacgtgtaataagaaaattgaaggcccacttagagaaactctagctttcttcagaatacaaggtcttggaattctcttttcaatgttaatgaatcgtagaaaagtttttgtttgttttttcatactacttatggcagagtccctgtcaacaaatgtaaaaacaataaaatacaccttggtcaaccaatatccttagaagcattgtattataaaattctcaagactcttgctgttatgtaattaatataccccatttcattttcttttccattataaacatgtattttataatctattccttgctgtaacatatagacttcttggccctagaaattaacttcttaattaataacacctaagatgttgtaatttccaaaatatttataagatgcttaattgaataaggaggaaacaaaaagagctttaaattctcaagaaatgcagaccaaatccaaatgctatgttaaaatacaaacattcaattcacattaaattatttattgaacaaattgaagataatgacatatgtttttattacaaagtcttccatcatcttatatcattgacacatattatgagacctgcatttgaagagtgaatagaaataagaaaatgttttcccaaccccacaaaaacagaaaaaaatatataattttataattatcttataaagccaaaagttttatgaattatactttttttattagttaaaaatgacagcataactaaggttaatttttatttctggaaacacaaaattaaggtagcacaacttcttgtagaactaacaagtctgaaagttcatggtatttcaatgcagtaaaataatatttctattgttagttttcagtttacctaatcaagtgacaaatataaaattcactacactgtatttttgttgacaaaagcatttcaccttacctagatttatataataaaaacaaattgtatccatcttccctttaaatatatgtacttcaaagtgatacaaagaattcacatgaaaacctttccctatgttttatctcctgaaaaaaaaaatgtatggaatagtatttttaaatcagatataatatccaatattatacatatcctaagaaattaaatcaattgtgtaaataatcattattaacttttgctctagccacggcatagaaagaaatgtacatctctattaatataaagtgatatcaataggaaagttcacatcttatgcatataccaaaaaaactaattaaagtatgttgcattttaaaagaattattcttatgccaaatttagtagtctagaaattgtttttttttttaaaaaaacaaattgatgattacttatccttttctaaaaggtgtctgtttgcttatacaatggaattggtaaaagtacacttatttataatagaatttcttggaacttaaaaaggagattcagaaaaacttattggatcaaattaaattgactagaacttcaagagaatactactttgaccaatactttaaaactataaaagtatttttaaacaaaaaagcacaatagacaataaaagaaatagaaaagttgagatactttaacaataatgacgatttctgtaggttgtaaaagtgtacatggtgcaattcccagagagcactacaagattcaaaagaaaaaaaaaacctgctaaaaaattctaaatgtctgtgctgtgaccaatctccatgaccaagttaccatgaaaagtaacattttgaagttattgagactgaggtttccttatggactccacccatgcccccacttgccagagccattcacttttttataggttatatgtttgttttcaacattcgtttttgaatggatgttgaaagttaggctaaaatttttacctaatttttctataatgattttaataacagtttcaatgctttaataatagatttaaagggcactttggcctttaaatattttcagagaataaactgtaatttctctctcaaacaagcctttcttattctgaaagatgtcttttatcttacaggaaagaaaaaaaatgagtttctaggagcctctccattaaactggcaggctgatttcatttctgatcccatacagtttctgctgtctttcccttggctgcaaaggtgatcaatcaggaatccaaactgccatcaatacccctttgtaactgcaatggctcaagtgaactccttccgtcttcaataactgacacagtgtcaacatctgcttccaataagattgtttctttttttccttgagtagagtaaatctgctgactgagatcgtaaatggttgtgtttttcccccttttaatgcggaagattttttccaccatattttccaactttccttcaagtcaagtaaaaataaaaaaaaattggataacttcaaaagaaatgttcttatcctaggtgccaaggaagtttgatatataactaaaaatataaactatggtgaatgaatgacactgtcctcataattttggacacagtaatttaaataaaattttggaacatgtaggaaaactgaattggacctacatgccactttaaggttaatttatttttccttcagaaatgacatactaaaaagtcagctaattaagaaacgtacatttatctcctataccaggtagaaggaacagttagtaggagaaaaagattctctttgcagtaatttcttacagaaaaacaatcatgtatctatttgattgctgcagaaacggatatggatgtgaagagaagagacctttgggagctcaatttaatgaactacttactcaactgataggcatctgtagtagctgttatttattgaacatctaatatgagctacatgattgatcgtgtgtgtgtgtgtctgtgtgtgtgtgtgtgtgtatgtgatttccaacttccagagcctgcctgttaggtattattccattttactcatgagataaataaatgaagccccaaaccacacataaacttttggctaaactagaatttagagaatggcctaacagccgagttcttttccattaattcattctgctttctatttatccctcattcaaaactctaacatatatactttcctttttccaccacttaacgccactgcccccatcggcttaattcagcaaacactatttaaagaagggacactcagtaaggaatagaatacaggttcttgaaacagtttctgatttccactttaaattataaatacaacattaaaccagatagcaaactcaaaagctagatagggtgacatattctgcaaatcttagaataggaatgggcaaatactttttgtataatgaataacaagcttctcaaaggcaactttcatgtcagtgcttagaatttgggttttttttttaaagtcttataaagttaaagaaataaatccctcaattatttgcaatccactcctcattttgcaaattttagagcaatcttagccatttttgcttaacaaaataatataaatactcttaagaagaaagaaaaaggagagcaaatagaggggaaagttaagagagggtgcttaactttcttaagaagacacattgatttctcaaaagtttagaggctctttcaaattaataatgagagacaaaataatctgttaggttcctgatttgtcaacattatgttgtttcttagctcccgatggtttattggtggaagcatagattctatttaaaataaacgagacaattttctagggtctacttcacagatatttagaaagcttgaataaaatctgatttgtaaaatcagacaaaagtcacctttgtctaaaggtggagtggttttaataaaattgtggaggcagatagtagccctcaataaaacagttcggaagcctctaagtccaacagcatcattttgatgtgaaaaaagaagagccagagaatgacaggattttaaacttggaatgaattcagaatattatgctaaattacaacccatcctcttttaggacttctaacagcaatatggtcctagaagacaattatagagacatgctcattctctttctatgtatatttttgatccactccctgggtggcagtgtaccccaaacacctaggtcctgttttctttttccttttgagacaggatcttgctctgttgcccaagctggagtacagtggtgcaatcacagctcactgcaagctgcaaactcaaactcccaggctcaaacgttcctccggactcagcctccagagtagctgggacaacaggtgtgccccacaatgcccaggtaatttttcagaaattttttgtagggatagggtctccctatgttgcctaggctgatcttgaactcctgggctcaagcaatcctcccgagcctctgcctcctataatactaggattacaggcatgagctgctgtgcccagcctgggtcctgttttcaaagagagagctcacttacaaatctttcctgtgtacagcagaaaccaggttcccaacatttctcagttcctcagagccaataaactttttgtctgacagttaccgggagaacacagagcaaagtctaaattcagggtgaagacatctaattaatgcccttcaattaaatttggtggaaaataagaaatggagctaggaataactactttccttttcctcttcattgggaaaatccaactgaatgatctgaatgagtttaacactactttcaaataaattacaaaggaagttaatgtattccgaaggtggatgtggatgaggcaaataaccctgtcagtcatcacacagggactgttgaatacttgcctttgaaaactcagaaggacacaaggcaaatccagatttataaattcactaaattttgtgctccatgtatttgggcaaattataaatgaaacaatcatatcaaatcaaattatggaccaaagtatagaaaatttaacctggctactcccaggaaatataagttcatattattagtgagtggaaggtatcttaaatttggaccccacaatggtaaaaatgtgcatattgtgtaaaagagagtctaggtaagaaacagcaaagtgcggagtgatgagagtacaaaagagtatatagatctgaagctcaaaagacggataggatataaatgaatacataaattacagccaaggaaaatatttgaaaattatctatgagaactctgcctagctgaacatgtcatgttcatgtctaaaaagttcgcatatatgatacgaacaattaaagatagaaagtggcatttcactgaacatactattttatgtgggtggagagaaaaatgggagaaatttgaaaaaacctctttataaagctaaaaaacttctctaatacactaacttttttacatgacatctctggaagcagttaatggaagaaatgaactttgcctttgaagtccagcagtatcaataactgttactttcataatcttaatcttctcctagcagtgtcttaatgataatttaaactttatttagatcctgagagctatatcaagttaaatcctcaaatttttaatttttagcccaatttaaattgtatataacctctggttttatttttaaattgtggcataaatttaaatcctaatatacactttattttgccctaaatttctttctaaaaaggaattaaatcaagtaaagccagatttaaacaaacaaaaaaagagacttgttaagttctgtgttgaaactattatatatagaactgtttgtttgtttgtttgtttgtttgtttagcttacagggataggtggcattataagaaagagctcgggctttgtaatttctctagtaccttcccagatattgttccttcaaatgcccttcaggaaaaacaaatcccacttaaaatatgactttttaaattgccatgaatgaataattaaaaacaagtaaaataagtcactggcactcataggtggcatggttaaatgcatttttttccttgtagttgtatataacctctggttccatttatcaaatttggatgggctagaaagagaattagtctcctctaggcaaactcttcatttgattgaaagtttatgccaactttcttattagtcaacctccaagttattctttgggagaaatcaaagcaataaaatatcatttctttagcacagtcattaaaaaaaaacttttcaagctatacatataattcaaaactaattgagctagcatggaattaaatctttactgagattcaatgtaaaaacaatactgcattggtttgactacggtatagctacttttgtaagaaggaaaaaaacaaaacatttgaggtaacctagaaagcacagacagagcatataatagacatcttagagataagcattttaaacatttttgccagtgcttctctgagagcaagttctttaaacagaactcaacaatttttacaattttaaaaaaaatacatccctcaaaaatagcccatcaatgctaaaccaaactttttgtatttctacaaaaatagatgcacatagagctacaaacttgtattcctgaaagaatgaacattttaatgtgtggttcatcctttcctgacaaggtggttggctaaaaaaaaaaatcaaaatgaaacaaaaacttagctatatattgataaaagcaagataacaaaaggagagagttgcacagttggcaaaggctcagatgaggaaataaacaaataaaaatgcttttcttcaatgtctgggacccactttgctttctcaagaaaggccgaaaaccagtcaactgcgtgacactttgtcttctccttctatgcctttcgtgtcctattgctgaatggaaaaacccgacagtatcttttcccagtgggcccttggatttatgctgcaacttaactcactaagattgtgtgtttcagtaccacggtgattccttactcttgtcttgatgctgtagacctgtatcgaatcccacgctgggcactatgtctactgttccatgaaaggctccagcccatgctgaggtagcagaggtgactgtagttggttctgtctttgtgatgtcacactggggagcaggaatcctggccgcatgcactgaaggcatcagcagaggcccataggatggatccagggcagagccagcaggagggtggtgatggtgatgatggtggcggtggcggtggtgcatgtgggcatgagggtggtggtgccgcatgtacacgtcatgcatatggctgtaggatgggctcacctgagatgtcaaaggataaggccaggactcagacacagcagggggaggggctgggccagtctgatgcaggttgtgtcccggccaaggactgggatcagctgcagaaaaggtgccagggggtccagtgacctggaagtcaggatgaactccccccaaacaaggtgcaggtgggggctggtaagagctggtccaaaaggaagttgggaaactattccgctggcttgagagagctgagctgtctcgccataggggggttagccccatcttgctttttgaaatggcagattctggatggagggtgatggcttggcccaaagctcttgagaagtgttcatccactactgacccaatgtctccctgctggccaggttggggcgccggctgatagtaggctgtggggcaggttgtcgctgccatggggttgggcagatactgggacgctccataaggctgggggtgatacatcacctccgcacaactcatggcagccggggcagtggcggcccccgagctgccgccgccgctctacgcgctggcgcgaggggcgcgggcgccgccgccgccgcagctgccgcctctgtcgctgctccagctgctactgcggcgaaggcgggtcctcggcggcctcgggctccgcgcggggcgcggggtcgggagggactggcaatcagcgggggcccatgcgcgggcaccttcatcttcagcccctccggatgttccctgccgcgcttatatagcggctcagggacgcagccgcccgctgcgccgctggggcattaccgcgtccggctcccgcgagggctgcggcgcccacggcagcgccagtcacagccacagcccaggcccgggtcgggcagccgtggggagcccagctccggtttgcatatac

SEQ ID NO: 18340 - RNA, 8515 nt, Homo sapiens
  source 1..8515: mol_type = other RNA
tgaagtaccagctactcgagaggctgaggcaggggaatcctttgaacccgggaggtggaggttggagtgagccgagatcgcgccactgcactccagcctgacgacagagcaagactccatcaaaacaaaacaaaacaaaacaaaacaaaaaaacaaaacagaacaaaaaccttgagatgaagagattattctggattacacagatgcagctattgtaatcacatgagtccttaaatatgtaagggagaggaagaagaggaagtcagtgatgtcatgtgagaaggtcttgaccaggttgctggatttgaagatggaaggaaactaagcaaaggactctagaagcagggaacagcaagattctctcttggaagcatccaggaaatgcctcctacattctgtagcccaccaagactaagatctttgctgaatgtctgactgacagagctgtaagataataaatttgtgttgttttaggccgttatcgttgtagtaatgtagtaatattttacagcagttctaaaaatctcattttgacaccacattctaaatatggtagacagttaaaaagcctgcgccaaattatttcatctgtaatgctggaaagtctattatttaaatgctgattttcagactttagtactttcacattaaagatacgtgtaataagaaaattgaaggcccacttagagaaactctagctttcttcagaatacaaggtcttggaattctcttttcaatgttaatgaatcgtagaaaagtttttgtttgttttttcatactacttatggcagagtccctgtcaacaaatgtaaaaacaataaaatacaccttggtcaaccaatatccttagaagcattgtattataaaattctcaagactcttgctgttatgtaattaatataccccatttcattttcttttccattataaacatgtattttataatctattccttgctgtaacatatagacttcttggccctagaaattaacttcttaattaataacacctaagatgttgtaatttccaaaatatttataagatgcttaattgaataaggaggaaacaaaaagagctttaaattctcaagaaatgcagaccaaatccaaatgctatgttaaaatacaaacattcaattcacattaaattatttattgaacaaattgaagataatgacatatgtttttattacaaagtcttccatcatcttatatcattgacacatattatgagacctgcatttgaagagtgaatagaaataagaaaatgttttcccaaccccacaaaaacagaaaaaaatatataattttataattatcttataaagccaaaagttttatgaattatactttttttattagttaaaaatgacagcataactaaggttaatttttatttctggaaacacaaaattaaggtagcacaacttcttgtagaactaacaagtctgaaagttcatggtatttcaatgcagtaaaataatatttctattgttagttttcagtttacctaatcaagtgacaaatataaaattcactacactgtatttttgttgacaaaagcatttcaccttacctagatttatataataaaaacaaattgtatccatcttccctttaaatatatgtacttcaaagtgatacaaagaattcacatgaaaacctttccctatgttttatctcctgaaaaaaaaaatgtatggaatagtatttttaaatcagatataatatccaatattatacatatcctaagaaattaaatcaattgtgtaaataatcattattaacttttgctctagccacggcatagaaagaaatgtacatctctattaatataaagtgatatcaataggaaagttcacatcttatgcatataccaaaaaaactaattaaagtatgttgcattttaaaagaattattcttatgccaaatttagtagtctagaaattgtttttttttttaaaaaaacaaattgatgattacttatccttttctaaaaggtgtctgtttgcttatacaatggaattggtaaaagtacacttatttataatagaatttcttggaacttaaaaaggagattcagaaaaacttattggatcaaattaaattgactagaacttcaagagaatactactttgaccaatactttaaaactataaaagtatttttaaacaaaaaagcacaatagacaataaaagaaatagaaaagttgagatactttaacaataatgacgatttctgtaggttgtaaaagtgtacatggtgcaattcccagagagcactacaagattcaaaagaaaaaaaaaacctgctaaaaaattctaaatgtctgtgctgtgaccaatctccatgaccaagttaccatgaaaagtaacattttgaagttattgagactgaggtttccttatggactccacccatgcccccacttgccagagccattcacttttttataggttatatgtttgttttcaacattcgtttttgaatggatgttgaaagttaggctaaaatttttacctaatttttctataatgattttaataacagtttcaatgctttaataatagatttaaagggcactttggcctttaaatattttcagagaataaactgtaatttctctctcaaacaagcctttcttattctgaaagatgtcttttatcttacaggaaagaaaaaaaatgagtttctaggagcctctccattaaactggcaggctgatttcatttctgatcccatacagtttctgctgtctttcccttggctgcaaaggtgatcaatcaggaatccaaactgccatcaatacccctttgtaactgcaatggctcaagtgaactccttccgtcttcaataactgacacagtgtcaacatctgcttccaataagattgtttctttttttccttgagtagagtaaatctgctgactgagatcgtaaatggttgtgtttttcccccttttaatgcggaagattttttccaccatattttccaactttccttcaagtcaagtaaaaataaaaaaaaattggataacttcaaaagaaatgttcttatcctaggtgccaaggaagtttgatatataactaaaaatataaactatggtgaatgaatgacactgtcctcataattttggacacagtaatttaaataaaattttggaacatgtaggaaaactgaattggacctacatgccactttaaggttaatttatttttccttcagaaatgacatactaaaaagtcagctaattaagaaacgtacatttatctcctataccaggtagaaggaacagttagtaggagaaaaagattctctttgcagtaatttcttacagaaaaacaatcatgtatctatttgattgctgcagaaacggatatggatgtgaagagaagagacctttgggagctcaatttaatgaactacttactcaactgataggcatctgtagtagctgttatttattgaacatctaatatgagctacatgattgatcgtgtgtgtgtgtgtctgtgtgtgtgtgtgtgtgtatgtgatttccaacttccagagcctgcctgttaggtattattccattttactcatgagataaataaatgaagccccaaaccacacataaacttttggctaaactagaatttagagaatggcctaacagccgagttcttttccattaattcattctgctttctatttatccctcattcaaaactctaacatatatactttcctttttccaccacttaacgccactgcccccatcggcttaattcagcaaacactatttaaagaagggacactcagtaaggaatagaatacaggttcttgaaacagtttctgatttccactttaaattataaatacaacattaaaccagatagcaaactcaaaagctagatagggtgacatattctgcaaatcttagaataggaatgggcaaatactttttgtataatgaataacaagcttctcaaaggcaactttcatgtcagtgcttagaatttgggttttttttttaaagtcttataaagttaaagaaataaatccctcaattatttgcaatccactcctcattttgcaaattttagagcaatcttagccatttttgcttaacaaaataatataaatactcttaagaagaaagaaaaaggagagcaaatagaggggaaagttaagagagggtgcttaactttcttaagaagacacattgatttctcaaaagtttagaggctctttcaaattaataatgagagacaaaataatctgttaggttcctgatttgtcaacattatgttgtttcttagctcccgatggtttattggtggaagcatagattctatttaaaataaacgagacaattttctagggtctacttcacagatatttagaaagcttgaataaaatctgatttgtaaaatcagacaaaagtcacctttgtctaaaggtggagtggttttaataaaattgtggaggcagatagtagccctcaataaaacagttcggaagcctctaagtccaacagcatcattttgatgtgaaaaaagaagagccagagaatgacaggattttaaacttggaatgaattcagaatattatgctaaattacaacccatcctcttttaggacttctaacagcaatatggtcctagaagacaattatagagacatgctcattctctttctatgtatatttttgatccactccctgggtggcagtgtaccccaaacacctaggtcctgttttctttttccttttgagacaggatcttgctctgttgcccaagctggagtacagtggtgcaatcacagctcactgcaagctgcaaactcaaactcccaggctcaaacgttcctccggactcagcctccagagtagctgggacaacaggtgtgccccacaatgcccaggtaatttttcagaaattttttgtagggatagggtctccctatgttgcctaggctgatcttgaactcctgggctcaagcaatcctcccgagcctctgcctcctataatactaggattacaggcatgagctgctgtgcccagcctgggtcctgttttcaaagagagagctcacttacaaatctttcctgtgtacagcagaaaccaggttcccaacatttctcagttcctcagagccaataaactttttgtctgacagttaccgggagaacacagagcaaagtctaaattcagggtgaagacatctaattaatgcccttcaattaaatttggtggaaaataagaaatggagctaggaataactactttccttttcctcttcattgggaaaatccaactgaatgatctgaatgagtttaacactactttcaaataaattacaaaggaagttaatgtattccgaaggtggatgtggatgaggcaaataaccctgtcagtcatcacacagggactgttgaatacttgcctttgaaaactcagaaggacacaaggcaaatccagatttataaattcactaaattttgtgctccatgtatttgggcaaattataaatgaaacaatcatatcaaatcaaattatggaccaaagtatagaaaatttaacctggctactcccaggaaatataagttcatattattagtgagtggaaggtatcttaaatttggaccccacaatggtaaaaatgtgcatattgtgtaaaagagagtctaggtaagaaacagcaaagtgcggagtgatgagagtacaaaagagtatatagatctgaagctcaaaagacggataggatataaatgaatacataaattacagccaaggaaaatatttgaaaattatctatgagaactctgcctagctgaacatgtcatgttcatgtctaaaaagttcgcatatatgatacgaacaattaaagatagaaagtggcatttcactgaacatactattttatgtgggtggagagaaaaatgggagaaatttgaaaaaacctctttataaagctaaaaaacttctctaatacactaacttttttacatgacatctctggaagcagttaatggaagaaatgaactttgcctttgaagtccagcagtatcaataactgttactttcataatcttaatcttctcctagcagtgtcttaatgataatttaaactttatttagatcctgagagctatatcaagttaaatcctcaaatttttaatttttagcccaatttaaattgtatataacctctggttttatttttaaattgtggcataaatttaaatcctaatatacactttattttgccctaaatttctttctaaaaaggaattaaatcaagtaaagccagatttaaacaaacaaaaaaagagacttgttaagttctgtgttgaaactattatatatagaactgtttgtttgtttgtttgtttgtttgtttagcttacagggataggtggcattataagaaagagctcgggctttgtaatttctctagtaccttcccagatattgttccttcaaatgcccttcaggaaaaacaaatcccacttaaaatatgactttttaaattgccatgaatgaataattaaaaacaagtaaaataagtcactggcactcataggtggcatggttaaatgcatttttttccttgtagttgtatataacctctggttccatttatcaaatttggatgggctagaaagagaattagtctcctctaggcaaactcttcatttgattgaaagtttatgccaactttcttattagtcaacctccaagttattctttgggagaaatcaaagcaataaaatatcatttctttagcacagtcattaaaaaaaaacttttcaagctatacatataattcaaaactaattgagctagcatggaattaaatctttactgagattcaatgtaaaaacaatactgcattggtttgactacggtatagctacttttgtaagaaggaaaaaaacaaaacatttgaggtaacctagaaagcacagacagagcatataatagacatcttagagataagcattttaaacatttttgccagtgcttctctgagagcaagttctttaaacagaactcaacaatttttacaattttaaaaaaaatacatccctcaaaaatagcccatcaatgctaaaccaaactttttgtatttctacaaaaatagatgcacatagagctacaaacttgtattcctgaaagaatgaacattttaatgtgtggttcatcctttcctgacaaggtggttggctaaaaaaaaaaatcaaaatgaaacaaaaacttagctatatattgataaaagcaagataacaaaaggagagagttgcacagttggcaaaggctcagatgaggaaataaacaaataaaaatgcttttcttcaatgtctgggacccactttgctttctcaagaaaggccgaaaaccagtcaactgcgtgacactttgtcttctccttctatgcctttcgtgtcctattgctgaatggaaaaacccgacagtatcttttcccagtgggcccttggatttatgctgcaacttaactcactaagattgtgtgtttcagtaccacggtgattccttactcttgtcttgatgctgtagacctgtatcgaatcccacgctgggcactatgtctactgttccatgaaaggctccagcccatgctgaggtagcagaggtgactgtagttggttctgtctttgtgatgtcacactggggagcaggaatcctggccgcatgcactgaaggcatcagcagaggcccataggatggatccagggcagagccagcaggagggtggtgatggtgatgatggtggcggtggcggtggtgcatgtgggcatgagggtggtggtgccgcatgtacacgtcatgcatatggctgtaggatgggctcacctgagatgtcaaaggataaggccaggactcagacacagcagggggaggggctgggccagtctgatgcaggttgtgtcccggccaaggactgggatcagctgcagaaaaggtgccagggggtccagtgacctggaagtcaggatgaactccccccaaacaaggtgcaggtgggggctggtaagagctggtccaaaaggaagttgggaaactattccgctggcttgagagagctgagctgtctcgccataggggggttagccccatcttgctttttgaaatggcagattctggatggagggtgatggcttggcccaaagctcttgagaagtgttcatccactactgacccaatgtctccctggaaataagtgaaaaggacacagcgagagttaaggtactccatctcggcaggctggtctttctcctcctcctcctcctcctcatcctcctcctcttgtttgctgggaagggtgacttccagagagtcctgcatcttgctgaataccgctaacttctgctggccaggttggggcgccggctgatagtaggctgtggggcaggttgtcgctgccatggggttgggcagatactgggacgctccataaggctgggggtgatacatcacctccgcacaactcatggcagccggggcag

SEQ ID NO: 18341 - RNA, 8910 nt, Homo sapiens
  source 1..8910: mol_type = other RNA
tgaagtaccagctactcgagaggctgaggcaggggaatcctttgaacccgggaggtggaggttggagtgagccgagatcgcgccactgcactccagcctgacgacagagcaagactccatcaaaacaaaacaaaacaaaacaaaacaaaaaaacaaaacagaacaaaaaccttgagatgaagagattattctggattacacagatgcagctattgtaatcacatgagtccttaaatatgtaagggagaggaagaagaggaagtcagtgatgtcatgtgagaaggtcttgaccaggttgctggatttgaagatggaaggaaactaagcaaaggactctagaagcagggaacagcaagattctctcttggaagcatccaggaaatgcctcctacattctgtagcccaccaagactaagatctttgctgaatgtctgactgacagagctgtaagataataaatttgtgttgttttaggccgttatcgttgtagtaatgtagtaatattttacagcagttctaaaaatctcattttgacaccacattctaaatatggtagacagttaaaaagcctgcgccaaattatttcatctgtaatgctggaaagtctattatttaaatgctgattttcagactttagtactttcacattaaagatacgtgtaataagaaaattgaaggcccacttagagaaactctagctttcttcagaatacaaggtcttggaattctcttttcaatgttaatgaatcgtagaaaagtttttgtttgttttttcatactacttatggcagagtccctgtcaacaaatgtaaaaacaataaaatacaccttggtcaaccaatatccttagaagcattgtattataaaattctcaagactcttgctgttatgtaattaatataccccatttcattttcttttccattataaacatgtattttataatctattccttgctgtaacatatagacttcttggccctagaaattaacttcttaattaataacacctaagatgttgtaatttccaaaatatttataagatgcttaattgaataaggaggaaacaaaaagagctttaaattctcaagaaatgcagaccaaatccaaatgctatgttaaaatacaaacattcaattcacattaaattatttattgaacaaattgaagataatgacatatgtttttattacaaagtcttccatcatcttatatcattgacacatattatgagacctgcatttgaagagtgaatagaaataagaaaatgttttcccaaccccacaaaaacagaaaaaaatatataattttataattatcttataaagccaaaagttttatgaattatactttttttattagttaaaaatgacagcataactaaggttaatttttatttctggaaacacaaaattaaggtagcacaacttcttgtagaactaacaagtctgaaagttcatggtatttcaatgcagtaaaataatatttctattgttagttttcagtttacctaatcaagtgacaaatataaaattcactacactgtatttttgttgacaaaagcatttcaccttacctagatttatataataaaaacaaattgtatccatcttccctttaaatatatgtacttcaaagtgatacaaagaattcacatgaaaacctttccctatgttttatctcctgaaaaaaaaaatgtatggaatagtatttttaaatcagatataatatccaatattatacatatcctaagaaattaaatcaattgtgtaaataatcattattaacttttgctctagccacggcatagaaagaaatgtacatctctattaatataaagtgatatcaataggaaagttcacatcttatgcatataccaaaaaaactaattaaagtatgttgcattttaaaagaattattcttatgccaaatttagtagtctagaaattgtttttttttttaaaaaaacaaattgatgattacttatccttttctaaaaggtgtctgtttgcttatacaatggaattggtaaaagtacacttatttataatagaatttcttggaacttaaaaaggagattcagaaaaacttattggatcaaattaaattgactagaacttcaagagaatactactttgaccaatactttaaaactataaaagtatttttaaacaaaaaagcacaatagacaataaaagaaatagaaaagttgagatactttaacaataatgacgatttctgtaggttgtaaaagtgtacatggtgcaattcccagagagcactacaagattcaaaagaaaaaaaaaacctgctaaaaaattctaaatgtctgtgctgtgaccaatctccatgaccaagttaccatgaaaagtaacattttgaagttattgagactgaggtttccttatggactccacccatgcccccacttgccagagccattcacttttttataggttatatgtttgttttcaacattcgtttttgaatggatgttgaaagttaggctaaaatttttacctaatttttctataatgattttaataacagtttcaatgctttaataatagatttaaagggcactttggcctttaaatattttcagagaataaactgtaatttctctctcaaacaagcctttcttattctgaaagatgtcttttatcttacaggaaagaaaaaaaatgagtttctaggagcctctccattaaactggcaggctgatttcatttctgatcccatacagtttctgctgtctttcccttggctgcaaaggtgatcaatcaggaatccaaactgccatcaatacccctttgtaactgcaatggctcaagtgaactccttccgtcttcaataactgacacagtgtcaacatctgcttccaataagattgtttctttttttccttgagtagagtaaatctgctgactgagatcgtaaatggttgtgtttttcccccttttaatgcggaagattttttccaccatattttccaactttccttcaagtcaagtaaaaataaaaaaaaattggataacttcaaaagaaatgttcttatcctaggtgccaaggaagtttgatatataactaaaaatataaactatggtgaatgaatgacactgtcctcataattttggacacagtaatttaaataaaattttggaacatgtaggaaaactgaattggacctacatgccactttaaggttaatttatttttccttcagaaatgacatactaaaaagtcagctaattaagaaacgtacatttatctcctataccaggtagaaggaacagttagtaggagaaaaagattctctttgcagtaatttcttacagaaaaacaatcatgtatctatttgattgctgcagaaacggatatggatgtgaagagaagagacctttgggagctcaatttaatgaactacttactcaactgataggcatctgtagtagctgttatttattgaacatctaatatgagctacatgattgatcgtgtgtgtgtgtgtctgtgtgtgtgtgtgtgtgtatgtgatttccaacttccagagcctgcctgttaggtattattccattttactcatgagataaataaatgaagccccaaaccacacataaacttttggctaaactagaatttagagaatggcctaacagccgagttcttttccattaattcattctgctttctatttatccctcattcaaaactctaacatatatactttcctttttccaccacttaacgccactgcccccatcggcttaattcagcaaacactatttaaagaagggacactcagtaaggaatagaatacaggttcttgaaacagtttctgatttccactttaaattataaatacaacattaaaccagatagcaaactcaaaagctagatagggtgacatattctgcaaatcttagaataggaatgggcaaatactttttgtataatgaataacaagcttctcaaaggcaactttcatgtcagtgcttagaatttgggttttttttttaaagtcttataaagttaaagaaataaatccctcaattatttgcaatccactcctcattttgcaaattttagagcaatcttagccatttttgcttaacaaaataatataaatactcttaagaagaaagaaaaaggagagcaaatagaggggaaagttaagagagggtgcttaactttcttaagaagacacattgatttctcaaaagtttagaggctctttcaaattaataatgagagacaaaataatctgttaggttcctgatttgtcaacattatgttgtttcttagctcccgatggtttattggtggaagcatagattctatttaaaataaacgagacaattttctagggtctacttcacagatatttagaaagcttgaataaaatctgatttgtaaaatcagacaaaagtcacctttgtctaaaggtggagtggttttaataaaattgtggaggcagatagtagccctcaataaaacagttcggaagcctctaagtccaacagcatcattttgatgtgaaaaaagaagagccagagaatgacaggattttaaacttggaatgaattcagaatattatgctaaattacaacccatcctcttttaggacttctaacagcaatatggtcctagaagacaattatagagacatgctcattctctttctatgtatatttttgatccactccctgggtggcagtgtaccccaaacacctaggtcctgttttctttttccttttgagacaggatcttgctctgttgcccaagctggagtacagtggtgcaatcacagctcactgcaagctgcaaactcaaactcccaggctcaaacgttcctccggactcagcctccagagtagctgggacaacaggtgtgccccacaatgcccaggtaatttttcagaaattttttgtagggatagggtctccctatgttgcctaggctgatcttgaactcctgggctcaagcaatcctcccgagcctctgcctcctataatactaggattacaggcatgagctgctgtgcccagcctgggtcctgttttcaaagagagagctcacttacaaatctttcctgtgtacagcagaaaccaggttcccaacatttctcagttcctcagagccaataaactttttgtctgacagttaccgggagaacacagagcaaagtctaaattcagggtgaagacatctaattaatgcccttcaattaaatttggtggaaaataagaaatggagctaggaataactactttccttttcctcttcattgggaaaatccaactgaatgatctgaatgagtttaacactactttcaaataaattacaaaggaagttaatgtattccgaaggtggatgtggatgaggcaaataaccctgtcagtcatcacacagggactgttgaatacttgcctttgaaaactcagaaggacacaaggcaaatccagatttataaattcactaaattttgtgctccatgtatttgggcaaattataaatgaaacaatcatatcaaatcaaattatggaccaaagtatagaaaatttaacctggctactcccaggaaatataagttcatattattagtgagtggaaggtatcttaaatttggaccccacaatggtaaaaatgtgcatattgtgtaaaagagagtctaggtaagaaacagcaaagtgcggagtgatgagagtacaaaagagtatatagatctgaagctcaaaagacggataggatataaatgaatacataaattacagccaaggaaaatatttgaaaattatctatgagaactctgcctagctgaacatgtcatgttcatgtctaaaaagttcgcatatatgatacgaacaattaaagatagaaagtggcatttcactgaacatactattttatgtgggtggagagaaaaatgggagaaatttgaaaaaacctctttataaagctaaaaaacttctctaatacactaacttttttacatgacatctctggaagcagttaatggaagaaatgaactttgcctttgaagtccagcagtatcaataactgttactttcataatcttaatcttctcctagcagtgtcttaatgataatttaaactttatttagatcctgagagctatatcaagttaaatcctcaaatttttaatttttagcccaatttaaattgtatataacctctggttttatttttaaattgtggcataaatttaaatcctaatatacactttattttgccctaaatttctttctaaaaaggaattaaatcaagtaaagccagatttaaacaaacaaaaaaagagacttgttaagttctgtgttgaaactattatatatagaactgtttgtttgtttgtttgtttgtttgtttagcttacagggataggtggcattataagaaagagctcgggctttgtaatttctctagtaccttcccagatattgttccttcaaatgcccttcaggaaaaacaaatcccacttaaaatatgactttttaaattgccatgaatgaataattaaaaacaagtaaaataagtcactggcactcataggtggcatggttaaatgcatttttttccttgtagttgtatataacctctggttccatttatcaaatttggatgggctagaaagagaattagtctcctctaggcaaactcttcatttgattgaaagtttatgccaactttcttattagtcaacctccaagttattctttgggagaaatcaaagcaataaaatatcatttctttagcacagtcattaaaaaaaaacttttcaagctatacatataattcaaaactaattgagctagcatggaattaaatctttactgagattcaatgtaaaaacaatactgcattggtttgactacggtatagctacttttgtaagaaggaaaaaaacaaaacatttgaggtaacctagaaagcacagacagagcatataatagacatcttagagataagcattttaaacatttttgccagtgcttctctgagagcaagttctttaaacagaactcaacaatttttacaattttaaaaaaaatacatccctcaaaaatagcccatcaatgctaaaccaaactttttgtatttctacaaaaatagatgcacatagagctacaaacttgtattcctgaaagaatgaacattttaatgtgtggttcatcctttcctgacaaggtggttggctaaaaaaaaaaatcaaaatgaaacaaaaacttagctatatattgataaaagcaagataacaaaaggagagagttgcacagttggcaaaggctcagatgaggaaataaacaaataaaaatgcttttcttcaatgtctgggacccactttgctttctcaagaaaggccgaaaaccagtcaactgcgtgacactttgtcttctccttctatgcctttcgtgtcctattgctgaatggaaaaacccgacagtatcttttcccagtgggcccttggatttatgctgcaacttaactcactaagattgtgtgtttcagtaccacggtgattccttactcttgtcttgatgctgtagacctgtatcgaatcccacgctgggcactatgtctactgttccatgaaaggctccagcccatgctgaggtagcagaggtgactgtagttggttctgtctttgtgatgtcacactggggagcaggaatcctggccgcatgcactgaaggcatcagcagaggcccataggatggatccagggcagagccagcaggagggtggtgatggtgatgatggtggcggtggcggtggtgcatgtgggcatgagggtggtggtgccgcatgtacacgtcatgcatatggctgtaggatgggctcacctgagatgtcaaaggataaggccaggactcagacacagcagggggaggggctgggccagtctgatgcaggttgtgtcccggccaaggactgggatcagctgcagaaaaggtgccagggggtccagtgacctggaagtcaggatgaactccccccaaacaaggtgcaggtgggggctggtaagagctggtccaaaaggaagttgggaaactattccgctggcttgagagagctgagctgtctcgccataggggggttagccccatcttgctttttgaaatggcagattctggatggagggtgatggcttggcccaaagctcttgagaagtgttcatccactactgacccaatgtctccctggaaataagtgaaaaggacacagcgagagttaaggtactccatctcggcaggctggtctttctcctcctcctcctcctcctcatcctcctcctcttgtttgctgggaagggtgacttccagagagtcctgcatcttgctgaataccgctaacttcttctgctggccaggttggggcgccggctgatagtaggctgtggggcaggttgtcgctgccatggggttgggcagatactgggacgctccataaggctgggggtgatacatcacctccgcacaactcatggcagccggggcagtggcggcccccgagctgccgccgccgctctacgcgctggcgcgaggggcgcgggcgccgccgccgccgcagctgccgcctctgtcgctgctccagctgctactgcggcgaaggcgggtcctcggcggcctcgggctccgcgcggggcgcggggtcgggagggactggcaatcagcgggggcccatgcgcgggcaccttcatcttcagcccctccggatgttccctgccgcgcttatatagcggctcagggacgcagccgcccgctgcgccgctggggcattaccgcgtccggctcccgcgagggctgcggcgcccacggcagcgccagtcacagccacagcccaggcccgggtcgggcagccgtggggagcccagctccggtttgcatatac

SEQ ID NO: 18342 - RNA, 988 nt, Homo sapiens
  source 1..988: mol_type = other RNA
tgaagtaccagctactcgagaggctgaggcaggggaatcggttgaacctgggaggcggaggttgcactgagctgagattgcgccactgcactcaaacctggcaacagagcgagactccatctcaaaaaaaaaagaaaaaaagaaaaaagaagacccatacaattctgatgtccctgtgctaattttatgcatgggatgctatacttgccctagttcattaatttcccaaggaaattagcacttataacccactcctctgattttaccaaaacaacaaagaattatacacacacacacatacacacacacagtcatgtacatttacatttaaaacattttatgagggataaaatatagtctttttctatcagtatgttcacacttcctggcctctcattgggaagctgtaagatgtccttcaataagatcctgaacacgcgacagaataatctcattagagctgctgcaattttctggaccatatggtgggtctatagtcaggaccccagccacacagagagtccttggagcgtctccctgttcagtgatggggatgtggttcttctcaagccatttctttaggctgttctttctctcttccagatcctctgggctgtatgctttgcagtctccagacgtgaacaaatgcatcagcttctccctcactctatggtccccttcattcatagtttcaacagtctgcacagcatgtcccataattccggtcacagacatgctgccatcttcaaggaagttcacaaggacaatattggcagagactgggtctgtagttaaaacccatcctttatactcattcttctcactggctgtcactcggacctctttgtaaatgtaatcttgccattctaaggggcctttcttcatccattcactcatgattgccacctggctaaatcagttaaaaaactcctcgcaactctgggtactcagcaaccatgctttgaggaaggatcgttgagcggagacc

SEQ ID NO: 18343 - RNA, 9017 nt, Homo sapiens
  source 1..9017: mol_type = other RNA
tgaagtaccagctactcgagaggctgaggcatgagaatcacttgaacctgggagatggaggttgcagtgagctgagatcacgccactcactccagcctgggcgacagaatgagactccgtctttcagctcttattccacccctgccttctggtggaggtggaggagggctactgcatctcacacttcagcctggtctcattcctcatcgtctcacaggattcacccttgccacttcagttcctggggtctcctgatgggaaacaggggtagcaaaggccagaaagaagcacagtggaggatggtttcctgaaccctccctgaaaaccaaagtggctgaaggaaacaacagcagacccatgagaagcaaggggcttttgcctgtgtgcagtggctcgcgcctgtaatcccagcactttgggaggccgaggcaggtggatcacttgaggtcaggagttcgagaccagcctggccaacatggtgaaacctcgtctcactaaaaatacaaaaattagccaggcgtggtagcacgcacctgtaatcccagctactcaggaggctaaggcaagagaatcgcttgagtccggaggcagaggttgcaggttgcagtcagtcaagatcgcaccactgtactccagcctgggcgacaaagtgagacacctcaaaaaaaaaaagaagaaaggggcttttgagaagtactgctaaaggaccacaattcccctcatggcacatgtaatctaaggaattcaatagaactttgttatttggaaattatttttgtttttcaacggagccctcagattaaaccacacggctgttttgtaatctcatgtactgaaagtttacaccttaaacacatctcttcttgacatgattcccataatcttatatatatgtggtcctcaggagaaagcagccagaattgccgtgggctttggcttaagaagacagaagggcaaagccacaggtggtaaagtcatgattgttgaaaggttctatatgataaagtgttaaatttcctcaaagtcataggattatggaactctcttcttcatgcttacctgcactttccaagttttatctgaacaatgaacatctagtaggtaaatcactaatgaagcttccttggtgctagggccacacttgagtgcgactgaatagtagatcctggggaaaagtatagtagaaccagagaatagaatgtcttacgtcagagtatattgaggtttccagcaacctaagcttgaatcagagtcccagcctctgtgagttggtctcaaggcccatggtccgtgctcgcttccagctccagcttcccgcttgggagaggccttggtttccatgagctgagcctctagattttggagaagattttctatggacaacacagacccaataacaaaagtactatgggaggaggctagatctgacttctaaacctgttcagttaccagagagatcagtaactccctaactcataaagggagggatggttaagcgaactagaaatatttagactgaagacttagaagtggccaactatcttcagaatggtagagggtaaacacctgggagagccgtaggggacagcccaaggatacccctccgtgaagttagagggaggcaagtttcttggtttaggaagattattccaacgaccagagatgcccatctgtgagtagactgcctcctgacaccgtcccaccttcaccagaagctggatctcactgcttcagatgctcagaaagcccttcagttatcaggaaagggctggaccaggtcatccttgccatctctctaccctgacctcccaattccacagtacagggctccttacaccgatttcagtttatttttatcagagcatgttcccttacagtccccaggctaacatgcagccccaaaaaaagcactatttgattcagtgaactgttgactgccagtcactgatccggaagtgtctgtttctagaactcagtgtttagccactgccacaccattcaggggctgctgccctcttgtggaaatgaagaatacgactgcttagaaaagaaattagatgcatttggaggctattgtctgtacacacattcccatcttaccttcccctaaaagcttaacattttagtgtgagccctaagcttaactttttagtgtgagccctgaagttcctaggtccagacagtcagggcctttggtttacattcacgctaccattctgtccaccaggatatggaactttagccacaatacaaaatcctggtttctagcgagattgacatttgtgaagaccattttgatgtgtggagtggcctttggatgttaacattgtgctgtgggaagagcactagcccacgcttaaagacccaggttccagctcgtgttctgccattcccttgtgaccctggacgagtcattttccagttgcatctgtggataaagggctacatgaccactggtacctggaacgctgtaatttattggatttagaaaatgctctaggagtttagagatgaaattctgtggagaacagtggcatatcacatgtgcactacttgtagctgctaaccacagcaaacagccacgggcttgattctaggttaggcaccctcaggctcctacaaaggagacctaggcattgttcatgtgtgcctcagcctcagggatagccatggtcagatgctttgcttttcccttaagtagaaatgtggcagactgttcagggagggtcccacaattcctagccttcacacgtgtctgaaaaacacttactaagttttctggacgagttttgccactagctcaggatacaaagctctgtgacccattagtgactggaagtgatttctcattgtttccaaatatcagtcacccgctccttgttaccactgcagggcttcatatggaggagggggcagctggggacaccacaaggtttgcctgagtgtgaggcaggtgttcaaccccaaactggaaaaatggcttgaaataaaactacagttggtagctgagtaaggaacatgactgtttcattttaaaaaaacccacttccttcttaagttttcccacaaaggataattttccctcaagaactgccttgccaagtatttcttgttgtagtctctaaatgctattttaaatgtagtctggggaactattttccgttggctcctaatactgaattaagctaacttgcccttatgatagtaacaaaaaatttcaagagcagaggatgctttgttgacctcagacgatttgtaccctcacacttgctgaaaataaaacatcttagcgaggtatttatgacattagtctgaaaacattttttcacttacatgaaatcttacacaatgaagtggcagtcaactgcaagaataaatgccgaatgagtcattttagttagcctgacctttgaggacacttggcttcgtagcaggtcttttcattaggtcttattctggtataaaaaggctccttcagaaaatgttttcactaaaaaataagttacaaactaacaagagtgctatataaccaacaattcctaagtattatgtaacagtaataaggcaaattcatcttaaaaaaggtttactagtaacagtggcctgctatggaccaggcactgtcctagtgttttacacacaaaaatctccagtccttacaacaaccctaaaaggcatacaagcagacaagcagactcgaatttgttgaatgattaagcaaggccatatagtactggtagaatccgaaagagaactcaggtctacccagttcttcttatgattaagctttttcctctccatctcctgaaagctgccttgaactggagtggggagaaatgggaggctccatgacagcatgccctgtgctttcaccaggtttctatatatacaggacatccatgtgagattttatgtgaaacaggttttggcttgcttcaagctgtatttcactatttagcaccctcttttgctcacagcagatgggctctagaggtcctgactaggcctgaaatgaggaacgctggggagcacctgtaggaatgctcagccctggatcaaactacagcatgctgtaagggacagtaccaaaaagaatgacaagggcagtgtggaagccatgtccctgcaacacaagggctggttcccaatcctggttatgatgctcagagctgtgaattgaagagatgtgtgattacatatttgcttgttgctttcctcgttagaagatagagagtcactttagttaaggtccatttaatttaacatttattttcattttatatccagatgtcacattttctacattaaaatataatcatgctgactcccccaacccccagccctcagagaaaaaagtgaagaactttacacaacatgaaagatggaatgcacggggtagggaagttgctattgcacccaagtaacaaagaacacagagagaccaacaggacgcatggcagaactgcatagaagatcgctcagggctcacgtcaggaaggcgcaggaattcagaaaactctaaagcttggaaatgctatcgtttgtgccacaaagattaccctgaaaaggtagagagaggtcaaaaagcagaaccaaattggggattttcaaaggctgctctctaacagagtttaaaatatccgtaaacataagtgcttctgctccctccccttgccttcagcatctggtaaacactttagaaacttaaaccactgttagcatgtcagaatgtagaaaggctgtaggtttttctttcttctcatcttgtaccccaaacaacaactctactggcaattgtaatcatgtgactcctctgcttggaaacccagtaaggatcaccaagacaaggggtctcactgctaccagacagataccagctgtgcaaaaagttgcaggattctgtgtattatttggagagggagagctgtaagacacaggaatcccaatacgtaagtactaaagagaaaaagaaaactcctttcactcatctattcattatataggaaagagcaaaaagacagtcaaaaccatctgcttcgagcagcagcacagcccagcaatacaggcataccaacaaaccgaaagcaaacactcaggaaagagcctcttggcccttctcaaaggagacttctctcagactggatcttgcccctaatgtagagaccaaagcattataacttcagagactggtactcttgagggagttgagaggtaaggtctaagagacccaaataacaagactgttatcaggtaactaactactccactatgtacaatacatacagcaataagaaaacgccactccatccctgcagcactttaaacatagcactgaggacccaggtagggggatattttaaggtctgttagcagtttaaaacgttgcaacactggcacaatatgttacctattctttgtttttaattacagggtaacatggtaaactccaacacaaaggtgggaaccgagagtgcaaaaggaataaagaaaacagaaccagtatttcacaagagcgcggagcaatgcagaagcagcagctaatgctttgcagagtctcgagggtaaaattcgctgagggtgctctgagggattctcttcagcatttctttggggaagattcggagtagctgccagccaatgtccaaagtctcaaagacagtgcgattttcgtaaggaccctgagcaatgaagttcctctcaaacttctgcagaaattccaagtagagaagatcatctgaggtaagggcttcttctccaacgacagctttcatggcttgcacatcctttccaatagcatagcacgcatatagctggttagatacatcggcatgatccttcctggtcatcccttctccaatagcagacttcattaaccgtgatagtgagggcagcacattgataggtggataaatctgtctgttgtgcagctgtctgtccacatagatctgcccctctgtaatgtagccagtcaagtctgggatggggtgagtgatatcatcattaggcatggttagaatagggatttgagtaatcgagccgtttctcccttccactcgcccagcgcgttcatatatcgtggctaaatctgtatacatgtaacctggaaaacctcgtcgaccaggtacctcttccctggctgctgaaacctgacagcaggtcaagcagaagagtatcatgcacgatattacaacaagcttgcttacaacatgtttgtttcaacatgccaaagtacaaagttgaaaatcccatcatgttcattttaaatactgtccttaagaatgatttagaaaaatctcccggcaacataaattcaaagtattctgtaacaaaaatgttgacaatggggcaccagaaggtttttgctaaaatcgtattgccataatgtaagttttcaaatagtttgctagaagaaaatctgtttgcaattttataaatcaaaggaagttaattttaaaacagaaaagattcttggttcacaagatttattccacgtggtggaactagccatatttatctaacctaatcccaaaaaggtcaaaagggaaggaaatgtacacgaggaatcatctgctgcgctttacaacattatttaacttaatcctcacagcaaccctatgaggaaggtgctacctccaattaacagttggaatcaagggtcagaaaaattaaacaatttctgaaggtcacaaagtcaggagtccattgcactgcacaaaataagaatggtgataaacgatctttcccttagagacatggataccagactataggtgtgcatgttcacctacaatcaactagaaccctaaagcattatgaaatccaacttctaagtgctactctgacatcttcaaaggagcgtgctacagcggtgctcctcacagcacggtctgcagaccaactgttatcaacatgcaatgatcacacagaaagcaagataagcatttagaaactttcagggcaatttggcagaataattttatgcctgttgaatctaacaattctaaaatctgcatttgtaaattatatatatagttaaaatttcacttttctaataactcaattttattgcattttacaaaagtattggtctgtgatggatgggggagaaaaactagtccttgactagagttagtctgaaacagcaatatagcagagtaagatatggtgagggcactgaaggaattttaagaagcctgtctcttcagaatctttttatgtgcttaaaaaagtaacttactcaaaatttcagtaatttgtattactgaacaaataccccaaaacttctaggggtaactgttataatctttctttaagaagcaggtctcgatctgtcacccagactggagggcagtggcacaatcatagcccaccgcagcctcaaattactggactcaagctatcctcccacctcagcctcctgagcaactaggattacaagtgtgtgtgccactacgcccagccaatatcttaatttttttgtggagaaagggtcttgctatgttacccaggctggtcttgaactcctgatcccaagtgaccctcctgccttggcttcccaaagtgctgggattacaggaatgagctaccgtgcccagcctgctagaatcttaatatttttcctaaataaacactgggttttctgaagaaaaaagtgctgaagagagtactgtgagagtagggtctttataaaatattaacatcattaaaaatggaattacaaaaaggtttaaaaattaatagtctggacagaaacagaacttcccgagagagtaactgaataaacagcttgaattatttactcccttttacaatcatttcttaatccatggagatagtgacagtatgataaacaggctaaccatttaaatcttaacctctaatcacttctaccaagttgacaaaaacgaagtagtttcctttctgatttattaaggcattctattaatatatgaacagtggaattaaaaaaccataaagaatgaaaacttgcaaagtgacaagttaaccctgaaaattaaccaattttgtttaactgagggaaaaacatgaacaacttacctctcgaagtgcttcagcataagaactcatgtctgttagaataaccaatacatgtttctcacattggtacgccagaaattcagctgtggttagagccaggcgaggagtgataattcgctcaatggttgggtcattagccaagttcaaaaagaggcagacattgtccattgagccattttcttcaaagtcagatttgaagaaccgggcagtttccatgtttacacccatagcagcaaatacaattgcaaaattttcctcactgtagtctactacatctttggatttctttaccaaaccagcctggcgacagatctgagctgcaatctcattgtgtggtagcccagcagcagagaagataggaattttctgccccctagcaatactgttcatcccatcgatggccgaaatgccagtctgaatcatttcctctgggtagattcgacattgagggttgattggctgacccatgatatcaaggaagtcttcggccagtacaacaggacctctgtcaatgggttttcccgatccattgaatacccgaccaagcatatcctcagacaccggtgttcggagaatatccccagtaaactcacaggacgttttcttagcatctatacctgaagtcccttcaaatacctgaactactgccttggaaccactaacttccagaacttgcccacttctctttgtgccatccggtaaggtcaaatggacaatttcagcatacctgggaaacttaacatgatctaagatcactagtggaccattgactccagatactgtcttgtatgtgaggcgaggctgggagaggtagttccgactgactgccagcgcctgctcccgagctcccaccgccggcccaccggtgggcacgggtagctcgggtgcggccccgttgacaatcccccgcatcgcccgcagcgccatcttgtctcctctgtcccgactggcccagcagc

SEQ ID NO: 18344 - RNA, 8549 nt, Homo sapiens
  source 1..8549: mol_type = other RNA
tgaagtaccagctactcgagaggctgaggcatgagaatcacttgaacctgggagatggaggttgcagtgagctgagatcacgccactcactccagcctgggcgacagaatgagactccgtctttcagctcttattccacccctgccttctggtggaggtggaggagggctactgcatctcacacttcagcctggtctcattcctcatcgtctcacaggattcacccttgccacttcagttcctggggtctcctgatgggaaacaggggtagcaaaggccagaaagaagcacagtggaggatggtttcctgaaccctccctgaaaaccaaagtggctgaaggaaacaacagcagacccatgagaagcaaggggcttttgcctgtgtgcagtggctcgcgcctgtaatcccagcactttgggaggccgaggcaggtggatcacttgaggtcaggagttcgagaccagcctggccaacatggtgaaacctcgtctcactaaaaatacaaaaattagccaggcgtggtagcacgcacctgtaatcccagctactcaggaggctaaggcaagagaatcgcttgagtccggaggcagaggttgcaggttgcagtcagtcaagatcgcaccactgtactccagcctgggcgacaaagtgagacacctcaaaaaaaaaaagaagaaaggggcttttgagaagtactgctaaaggaccacaattcccctcatggcacatgtaatctaaggaattcaatagaactttgttatttggaaattatttttgtttttcaacggagccctcagattaaaccacacggctgttttgtaatctcatgtactgaaagtttacaccttaaacacatctcttcttgacatgattcccataatcttatatatatgtggtcctcaggagaaagcagccagaattgccgtgggctttggcttaagaagacagaagggcaaagccacaggtggtaaagtcatgattgttgaaaggttctatatgataaagtgttaaatttcctcaaagtcataggattatggaactctcttcttcatgcttacctgcactttccaagttttatctgaacaatgaacatctagtaggtaaatcactaatgaagcttccttggtgctagggccacacttgagtgcgactgaatagtagatcctggggaaaagtatagtagaaccagagaatagaatgtcttacgtcagagtatattgaggtttccagcaacctaagcttgaatcagagtcccagcctctgtgagttggtctcaaggcccatggtccgtgctcgcttccagctccagcttcccgcttgggagaggccttggtttccatgagctgagcctctagattttggagaagattttctatggacaacacagacccaataacaaaagtactatgggaggaggctagatctgacttctaaacctgttcagttaccagagagatcagtaactccctaactcataaagggagggatggttaagcgaactagaaatatttagactgaagacttagaagtggccaactatcttcagaatggtagagggtaaacacctgggagagccgtaggggacagcccaaggatacccctccgtgaagttagagggaggcaagtttcttggtttaggaagattattccaacgaccagagatgcccatctgtgagtagactgcctcctgacaccgtcccaccttcaccagaagctggatctcactgcttcagatgctcagaaagcccttcagttatcaggaaagggctggaccaggtcatccttgccatctctctaccctgacctcccaattccacagtacagggctccttacaccgatttcagtttatttttatcagagcatgttcccttacagtccccaggctaacatgcagccccaaaaaaagcactatttgattcagtgaactgttgactgccagtcactgatccggaagtgtctgtttctagaactcagtgtttagccactgccacaccattcaggggctgctgccctcttgtggaaatgaagaatacgactgcttagaaaagaaattagatgcatttggaggctattgtctgtacacacattcccatcttaccttcccctaaaagcttaacattttagtgtgagccctaagcttaactttttagtgtgagccctgaagttcctaggtccagacagtcagggcctttggtttacattcacgctaccattctgtccaccaggatatggaactttagccacaatacaaaatcctggtttctagcgagattgacatttgtgaagaccattttgatgtgtggagtggcctttggatgttaacattgtgctgtgggaagagcactagcccacgcttaaagacccaggttccagctcgtgttctgccattcccttgtgaccctggacgagtcattttccagttgcatctgtggataaagggctacatgaccactggtacctggaacgctgtaatttattggatttagaaaatgctctaggagtttagagatgaaattctgtggagaacagtggcatatcacatgtgcactacttgtagctgctaaccacagcaaacagccacgggcttgattctaggttaggcaccctcaggctcctacaaaggagacctaggcattgttcatgtgtgcctcagcctcagggatagccatggtcagatgctttgcttttcccttaagtagaaatgtggcagactgttcagggagggtcccacaattcctagccttcacacgtgtctgaaaaacacttactaagttttctggacgagttttgccactagctcaggatacaaagctctgtgacccattagtgactggaagtgatttctcattgtttccaaatatcagtcacccgctccttgttaccactgcagggcttcatatggaggagggggcagctggggacaccacaaggtttgcctgagtgtgaggcaggtgttcaaccccaaactggaaaaatggcttgaaataaaactacagttggtagctgagtaaggaacatgactgtttcattttaaaaaaacccacttccttcttaagttttcccacaaaggataattttccctcaagaactgccttgccaagtatttcttgttgtagtctctaaatgctattttaaatgtagtctggggaactattttccgttggctcctaatactgaattaagctaacttgcccttatgatagtaacaaaaaatttcaagagcagaggatgctttgttgacctcagacgatttgtaccctcacacttgctgaaaataaaacatcttagcgaggtatttatgacattagtctgaaaacattttttcacttacatgaaatcttacacaatgaagtggcagtcaactgcaagaataaatgccgaatgagtcattttagttagcctgacctttgaggacacttggcttcgtagcaggtcttttcattaggtcttattctggtataaaaaggctccttcagaaaatgttttcactaaaaaataagttacaaactaacaagagtgctatataaccaacaattcctaagtattatgtaacagtaataaggcaaattcatcttaaaaaaggtttactagtaacagtggcctgctatggaccaggcactgtcctagtgttttacacacaaaaatctccagtccttacaacaaccctaaaaggcatacaagcagacaagcagactcgaatttgttgaatgattaagcaaggccatatagtactggtagaatccgaaagagaactcaggtctacccagttcttcttatgattaagctttttcctctccatctcctgaaagctgccttgaactggagtggggagaaatgggaggctccatgacagcatgccctgtgctttcaccaggtttctatatatacaggacatccatgtgagattttatgtgaaacaggttttggcttgcttcaagctgtatttcactatttagcaccctcttttgctcacagcagatgggctctagaggtcctgactaggcctgaaatgaggaacgctggggagcacctgtaggaatgctcagccctggatcaaactacagcatgctgtaagggacagtaccaaaaagaatgacaagggcagtgtggaagccatgtccctgcaacacaagggctggttcccaatcctggttatgatgctcagagctgtgaattgaagagatgtgtgattacatatttgcttgttgctttcctcgttagaagatagagagtcactttagttaaggtccatttaatttaacatttattttcattttatatccagatgtcacattttctacattaaaatataatcatgctgactcccccaacccccagccctcagagaaaaaagtgaagaactttacacaacatgaaagatggaatgcacggggtagggaagttgctattgcacccaagtaacaaagaacacagagagaccaacaggacgcatggcagaactgcatagaagatcgctcagggctcacgtcaggaaggcgcaggaattcagaaaactctaaagcttggaaatgctatcgtttgtgccacaaagattaccctgaaaaggtagagagaggtcaaaaagcagaaccaaattggggattttcaaaggctgctctctaacagagtttaaaatatccgtaaacataagtgcttctgctccctccccttgccttcagcatctggtaaacactttagaaacttaaaccactgttagcatgtcagaatgtagaaaggctgtaggtttttctttcttctcatcttgtaccccaaacaacaactctactggcaattgtaatcatgtgactcctctgcttggaaacccagtaaggatcaccaagacaaggggtctcactgctaccagacagataccagctgtgcaaaaagttgcaggattctgtgtattatttggagagggagagctgtaagacacaggaatcccaatacgtaagtactaaagagaaaaagaaaactcctttcactcatctattcattatataggaaagagcaaaaagacagtcaaaaccatctgcttcgagcagcagcacagcccagcaatacaggcataccaacaaaccgaaagcaaacactcaggaaagagcctcttggcccttctcaaaggagacttctctcagactggatcttgcccctaatgtagagaccaaagcattataacttcagagactggtactcttgagggagttgagaggtaaggtctaagagacccaaataacaagactgttatcaggtaactaactactccactatgtacaatacatacagcaataagaaaacgccactccatccctgcagcactttaaacatagcactgaggacccaggtagggggatattttaaggtctgttagcagtttaaaacgttgcaacactggcacaatatgttacctattctttgtttttaattacagggtaacatggtaaactccaacacaaaggtgggaaccgagagtgcaaaaggaataaagaaaacagaaccagtatttcacaagagcgcggagcaatgcagaagcagcagctaatgctttgcagagtctcgagggtaaaattcgctgagggtgctctgagggattctcttcagcatttctttggggaagattcggagtagctgccagccaatgtccaaagtctcaaagacagtgcgattttcgtaaggaccctgagcaatgaagttcctctcaaacttctgcagaaattccaagtagagaagatcatctgaggtaagggcttcttctccaacgacagctttcatggcttgcacatcctttccaatagcatagcacgcatatagctggttagatacatcggcatgatccttcctggtcatcccttctccaatagcagacttcattaaccgtgatagtgagggcagcacattgataggtggataaatctgtctgttgtgcagctgtctgtccacatagatctgcccctctgtaatgtagccagtcaagtctgggatggggtgagtgatatctaccagaggaagacagttggcattaagcatggcatctttaggttatgagttttaaagcggccatctctcagaaccaaacccacaaaaagtccctctgtactacctgtaacattacttagaagagtgttcttagagtcattttctgtgatgctgccaatgttctgtgtctgtgctgtgcagtacggtagccattagccaaatgtggctatctaacacttgaaacgtggctaacaaaactgaaaaacttaatttcaattatttcagttaacttgaacttaaacagccaaatgtggctagcggcaaccatactggccagtttagtttggttgcagcagttagacatgtgttggctctatgaggtaaactggctgcattcattaaaaatactctctcccctaggtaagcgctctcccctctcaatataagtaaagtttcattttaaacccaaagttcccttatagaaatttgccaacctgatgtatactaagaacattcttagttcataagctatgtcggatggatacacaacatttcaccatgcaaaacgcaggcatatagacaagtaaacaacactacacaggctgcaccaaaaaggtcacacaaagcaacacatttccaaatctgttaaattacatcattttgtagctactcccttggaacaaatcattttcacgtcagaggcagtacagagtaacagtgtgagttatgaactcaaactgggtcctaaatctatcacttgctaatctcaacaaatcatttgacctccctgtgcctcaaacagcatctgcctcaaagttgctatgaggagcaaatgagtgaatatttataaagcactcagaacagtgctcaattacagtaagtaataacttaccatattttgtcaaagtgttgttcaaaaactgaaataaggacaaagaggcaacacaggagaggaattctgaatagtcgtaccccatcctgggcacacacacagacaggcattggaaagtcatttttaaccagcccttggttaaaaaaatctgtctctcagttttgtggagtttcccacttgtactcctcatgtggcactgaacatggccatgttaaattaccggtgcacacacataaaaaacatccccaattagactgagtaacttacattaagtagagaccataaattcttttcaaaaattctttacatttagaacagtgtcctgcaaacagcaggcactcaatagtacctaataaagttaaaaacttaaattatgaagaaaattgcttttcctccacaataggataataactgtgggtaattttcaaatgaaaaatgttttatttaggcaaataaccaagataaactcttaggggatgtgttctcaaaataacttcaactcgaaaaggtagatgggtcttctctctctttaaaatgattaggtgtgttataatccaaataccaaaacttaccatcattaggcatggttagaatagggatttgagtaatcgagccgtttctcccttccactcgcccagcgcgttcatatatcgtggctaaatctgtatacatgtaacctggaaaacctcgtcgaccaggtacctcttccctggctgctgaaacctctcgaagtgcttcagcataagaactcatgtctgttagaataaccaatacatgtttctcacattggtacgccagaaattcagctgtggttagagccaggcgaggagtgataattcgctcaatggttgggtcattagccaagttcaaaaagaggcagacattgtccattgagccattttcttcaaagtcagatttgaagaaccgggcagtttccatgtttacacccatagcagcaaatacaattgcaaaattttcctcactgtagtctactacatctttggatttctttaccaaaccagcctggcgacagatctgagctgcaatctcattgtgtggtagcccagcagcagagaagataggaattttctgccccctagcaatactgttcatcccatcgatggccgaaatgccagtctgaatcatttcctctgggtagattcgacattgagggttgattggctgacccatgatatcaaggaagtcttcggccagtacaacaggacctctgtcaatgggttttcccgatccattgaatacccgaccaagcatatcctcagacaccggtgttcggagaatatccccagtaaactcacaggacgttttcttagcatctatacctgaagtcccttcaaatacctgaactactgccttggaaccactaacttccagaacttgcccacttctctttgtgccatccggtaaggtcaaatggacaatttcagcatacctgggaaacttaacatgatctaagatcactagtggaccattgactccagatactgtcttgtatgtgaggcgaggctgggagaggtagttccgactgactgccagcgcctgctcccgagctcccaccgccggcccaccggtgggcacgggtagctcgggtgcggccccgttgacaatcccccgcatcgcccgcagcgccatcttgtctcctctgtcccgactggcccagcagc

SEQ ID NO: 18345 - RNA, 455 nt, Homo sapiens
  source 1..455: mol_type = other RNA
tgaagtaccagctactcgagaggctgaggtgagaggactgcttgaagccgagttcgataccagcctggacgacatcatgagactctagctctgtaatctcagcactttgggaggccaaggtgagaggatctcttgagcccaggagttccagaccagcatggacgacatagggcaatctgtgatagtcctggtcccagctcctggaaagctctttgctcttagaagatctccctttcctccagcaaaatgtcatctcgccaggtgccatggcttgtacctgtaatcacagctactcaggaggctgaagcaggaggatcactggaggccaggagttggagaccagcctggatgacagagggagatcccatctctgtctatagtttgatgatagcctcttgaggataggggctttgtcttattcttatgggaccccagtgcttagaatagtgtcttat

SEQ ID NO: 18346 - RNA, 3301 nt, Homo sapiens
  source 1..3301: mol_type = other RNA
tgaagtaccagctactcgagaggctgaggtgagaggattgcttaagccctggaggttgaggctgcagtgagccatgatcatgccactgcactccagcctgggtgacagagaggccctgtctcaacaaataaacaaatgaaatgaaacaaaacaaaacaaaaatacccatccctaaatagcatccagctctctgtgtgcctttctctttgatagtttatgactagacttccttaatcagctacaaaggaaggcttaaagaaattatggaaatacctagccacaaagaacactttagagtggaggagtcagagagaaggagagtgcgagaggaatggacgtttcctcccttctttttggatgggcttaaatcatggatagtgtctcacattgaatggaagtgggaacaaagcttggacataaaggagatggggtggaaagcagcagtgggagctggaagggaactcttggctggccagcctgcacaaaggggagcagcacatttcacagaaaaatacatttatgcagctggccaggaggatgctgatggtctgagagtgaattgcagaaaatgtgtgcatgtgcccttagcatgggtgaggctgagctaagtgagtctacccttcctttttaaaagctctaatattgtcccctaaccaaaagatatgggaatcttagaatgacatttgcactttcagttatgttagttattacaagcacacaggccttacctactcccagaaagcatgcaaattatcttaccaagagatttcataacataatacagttagaatatattaaaatgagattcataaccgctaaatgtgaggcaaagctaattgtaacaagaacctcaaataaaataggaatctgggttttacctttgtgtttcctagaagccacagcaaaaagataaaataagggaacctacagctcataaaaggtagcagacaattttgactggaatctctttctcctcctctaaagtatgttagagtctctcctatgcatgggtggggtctgtgatgtttgcattggacctgcaaaatcatccagccctgtttcttcatttttcagggatgcagatggagattcagaggtgacagtgatgtgcccaaggacacaggtgtcagaagtgggatttcctttctcacggtaccaaatggccagcttggtttgtcagcctgttgtcttatcccaccatgactgtggtcagatgaaaaaactcggctcttgcttcatctgttccctgcagctgcagtccgtttggatagactcagacttaggggtggacgtgaggcagggctcatgggcagtcctcagctgtggcaatgacacccacacaccaacagctgcatggtgacttagctcccttttgggctccagcggctcctctagctctgagatactgagggttcttccagggaagcctgcactggggcagaagcctctacatgggcctgtgcctaggatggggctaatgtcggccatggtgtcggggaagggcgccaagcccactgggtggggcgatgcaggctgggcagggctgctctttcccagcctccttccagagtgggccgtttgcagagtagctgggctgccttcttgttgtgaggatgtggccacttctgcagtggcgctgaagtacaacgtggaactctgctgtccttcccctcctctctgctgcccacctgtccccttcccctgtgtcccagaaacagcgtcagctccttcctttggggtgccctccccctgcgtggctgctgggttctgggtaggtgcttcatcctgctgatcgctggcaaaagatacgtaacttgaggtttccaatgggtcggcctctgctttagggacaccttcaaacgcagagctgttctctaaggttgaggggtcacgggatgaggatgggagctcttgctgggcagacaaggcctttctctgcaggtagtcctgttgactcaacccccatgcaggtggacaataggcaggactgttatctccaaaggcggcattgatcttagacacatttcctgtttttagggcaagtttcacccacagccagtggtgatgactgaggaaagagtcctccacagcaacctgggtccccagcccagcctctggggggacctgctcaggggtagggggcttccctaaaatggttggttcataacttgccccttggcatgagcctgagctctcggttctcttcccagctagatctgtggcccggggagaatctcttctctctgttttatcacctcctgcaatgccacaggacttccttaggcagccctgccagatgtctgtggattttggatgcagcaggctgtaataaattaccagtgagacactgccaatcagaaatccagacaggaccccagctatggtctgcaggctggtccacgatgccccctggagaaagtcggtggccaacagcaacaggatgatgttctccaacagcatgaccatgtagaacgtgaccatcctatttctagaagggctgtcccagaagctgaggtagcagaggatgtacacggcccccacgagcaggttgaacagcctccagtggcaggtgctgtcgatgatgtcactctgctgggcgacaagccagaatgtcatcaccagccagtgggcacctgcaaccacaaaaacccaaaagtggtaggctttgtagaacagaaccagactcagcacgcgggttcccaacatgcccatcctccagagctgctggcagaagagggcggcccatggcatggccaggtggcctggcttcatgaagcccatgaagcgagtgtaggacaccagtgcccaggagagtgaggaccaggaaaacagggtgctcacccctggcacaatatctgtgaagtctgaggctagaaaaacatatgtctgaagcagcaggtggggcccagtctgcagcagggcctccaagagtcgaagggccgacaggtcggcctcctgcagctgcagccagcctcggtggggagcctccagttccttctgcagactggtcagtgcagcgtcccagtgccgcttccaaacaccaagctgtaggaggtgcagcatcatcaaggagcaatgccctggatgcccgtctgctcggaaccacaggtagctcagggcctggaccaagaacccgggcaggaggacagcaagggccagccacccccacagaagccgtcctgtggtgaagtagtaagccacggtgtaaaggcgcgcgctctgctcggccgcctgcagcagggccgagagccccaggagcctcgcgtgcatcttccgtgccgaccccgcagcctgcgcccgc

SEQ ID NO: 18347 - RNA, 3439 nt, Homo sapiens
  source 1..3439: mol_type = other RNA
tgaagtaccagctactcgagaggctgaggtgagaggattgcttaagccctggaggttgaggctgcagtgagccatgatcatgccactgcactccagcctgggtgacagagaggccctgtctcaacaaataaacaaatgaaatgaaacaaaacaaaacaaaaatacccatccctaaatagcatccagctctctgtgtgcctttctctttgatagtttatgactagacttccttaatcagctacaaaggaaggcttaaagaaattatggaaatacctagccacaaagaacactttagagtggaggagtcagagagaaggagagtgcgagaggaatggacgtttcctcccttctttttggatgggcttaaatcatggatagtgtctcacattgaatggaagtgggaacaaagcttggacataaaggagatggggtggaaagcagcagtgggagctggaagggaactcttggctggccagcctgcacaaaggggagcagcacatttcacagaaaaatacatttatgcagctggccaggaggatgctgatggtctgagagtgaattgcagaaaatgtgtgcatgtgcccttagcatgggtgaggctgagctaagtgagtctacccttcctttttaaaagctctaatattgtcccctaaccaaaagatatgggaatcttagaatgacatttgcactttcagttatgttagttattacaagcacacaggccttacctactcccagaaagcatgcaaattatcttaccaagagatttcataacataatacagttagaatatattaaaatgagattcataaccgctaaatgtgaggcaaagctaattgtaacaagaacctcaaataaaataggaatctgggttttacctttgtgtttcctagaagccacagcaaaaagataaaataagggaacctacagctcataaaaggtagcagacaattttgactggaatctctttctcctcctctaaagtatgttagagtctctcctatgcatgggtggggtctgtgatgtttgcattggacctgcaaaatcatccagccctgtttcttcatttttcagggatgcagatggagattcagaggtgacagtgatgtgcccaaggacacaggtgtcagaagtgggatttcctttctcacggtaccaaatggccagcttggtttgtcagcctgttgtcttatcccaccatgactgtggtcagatgaaaaaactcggctcttgcttcatctgttccctgcagctgcagtccgtttggatagactcagacttaggggtggacgtgaggcagggctcatgggcagtcctcagctgtggcaatgacacccacacaccaacagctgcatggtgacttagctcccttttgggctccagcggctcctctagctctgagatactgagggttcttccagggaagcctgcactggggcagaagcctctacatgggcctgtgcctaggatggggctaatgtcggccatggtgtcggggaagggcgccaagcccactgggtggggcgatgcaggctgggcagggctgctctttcccagcctccttccagagtgggccgtttgcagagtagctgggctgccttcttgttgtgaggatgtggccacttctgcagtggcgctgaagtacaacgtggaactctgctgtccttcccctcctctctgctgcccacctgtccccttcccctgtgtcccagaaacagcgtcagctccttcctttggggtgccctccccctgcgtggctgctgggttctgggtaggtgcttcatcctgctgatcgctggcaaaagatacgtaacttgaggtttccaatgggtcggcctctgctttagggacaccttcaaacgcagagctgttctctaaggttgaggggtcacgggatgaggatgggagctcttgctgggcagacaaggcctttctctgcaggtagtcctgttgactcaacccccatgcaggtggacaataggcaggactgttatctccaaaggcggcattgatcttagacacatttcctgtttttagggcaagtttcacccacagccagtggtgatgactgaggaaagagtcctccacagcaacctgggtccccagcccagcctctggggggacctgctcaggggtagggggcttccctaaaatggttggttcataacttgccccttggcatgagcctgagctctcggttctcttcccagctagatctgtggcccggggagaatctcttctctctgttttatcacctcctgcaatgccacaggacttccttaggcagccctgccagatgtctgtggattttggatgcagcaggctgtaataaattaccagtgagacactgccaatcagaaatccagacaggaccccagctatggtctgcaggctggtccacgatgccccctggagaaagtcggtggccaacagcaacaggatgatgttctccaacagcatgaccatgtagaacgtgaccatcctatttctagaagggctgtcccagaagctgaggtagcagaggatgtacacggcccccacgagcaggttgaacagcctccagtggcaggtgctgtcgatgatgtcactctgctgggcgacaagccagaatgtcatcaccagccagtgggcacctgcaaccacaaaaacccaaaagtggtaggctttgtagaacagaaccagactcagcacgcgggttcccaacatgcccatcctccagagctgctggcagaagagggcggcccatggcatggccaggtggcctggcttcatgaagcccatgaagcgagtgtaggacaccagtgcccaggagagtgaggaccaggaaaacagggtgctcacccctggcacaatatctgtgaagtctgaggctagaaaaacatatgtctgaagcagcaggtggggcccagtctgcagcagggcctccaagagtcgaagggccgacaggtcggcctcctgcagctgcagccagcctcggtggggagcctccagttccttctgcagactggtcagtgcagcgtcccagtgcctttagagtttaccttaactttccttttgacaaccttgaactttcactaaagaaaaattgctaaaccaaggtgcatgctaaggatgagataggccttcttctgtcatctcatgctgcatttacaagtggatttgtgggcgcttccaaacaccaagctgtaggaggtgcagcatcatcaaggagcaatgccctggatgcccgtctgctcggaaccacaggtagctcagggcctggaccaagaacccgggcaggaggacagcaagggccagccacccccacagaagccgtcctgtggtgaagtagtaagccacggtgtaaaggcgcgcgctctgctcggccgcctgcagcagggccgagagccccaggagcctcgcgtgcatcttccgtgccgaccccgcagcctgcgcccgc

SEQ ID NO: 18348 - RNA, 3277 nt, Homo sapiens
  source 1..3277: mol_type = other RNA
tgaagtaccagctactcgagaggctgaggtgggagaattgcttgaatcccagaggtggaggttgcagtgagccaagattgcaccactgcactccagccttggggacagagaaagaaagagagaaagagagacagagagagtgaccaagacagaccacacacccaggtctcggatggtaaggggctgaagcggctgctcttctgcctttctgctgctcgtggttcagtctgttcagattgtttcctgttgttaattgcggccccattccatgtctcagtccaaactgcgagagcaacatgtcattgcctgggccttccagccaggcaggccacacaggtcagaagtggctggctagcctggggatgaccacccccttctcggaccaagatgggccatgggaggggcaggaattcctttgagaggagacctaggggtgtggggtctgggcaggtaaggtaagtgatacctactagttgccttgttgcttttcccattttccccaacttttcagaaaaatgctggcctttatagcgacatcaggatgatggtagctaatattctattgagtgtttgctgtgtgccaggcactgtgctgtgctcagcacgtgttacaggcattaactgtgttcccaccttggctcagagaggatttggtcacttgccagggtcccatatctagctaatgatgccaagcttctactccgtcactttaagttagataaagtgtatgtggcagaattcccaagtcccagaggactgctccattgggagtagggaagacccagagcacggccagccaggctggtaagcagttgccaggtggcaggaagtggcttacactaagggttgaagcaaggcagagaagggaaaatgtgagcatttcaggacaaaacagaaacaaacaccaacatttcaggaatgagaagccagaagagagggaaggtttggccaaaggactggaaaggggcaagaaaatgaaatatgaaccaggaagctataggcaatcagcagaagtccacagctaatttgcataataaaaggaaaagtcatcttgttggaatttgtggtggtggctgcctagatttgaaattgtatcctataatttgccccatttccagtgagaaccagcgtaaaacatttctagaacaaacagtatattgcacaaggatagatttacaacaaaaactagtttttctaagacttgaagccttctgtcttttatcacagggggacccaggaagcccaatgatgtgccagctacagcagttcgatctgtgggttctgagaggagtcctgaacttcggtggtgagacgtgccctggcctgtttctgtacaccaaggtggaagactacagcaaatggatcacatccaaggctgagagggccggccctcccctgtcctcactccaccactgggaaaagttgatttctttctcccaccatggaccaaatgccaccatgacacagaagacatattctgattctgaactgggccatgttggatcatacttgcagggacaaagaaggaccatcacgcattcacgactaggaaacagctctagagatagtctagatgttagggagaaggatgtaaaggaatcaggcaggtctcctgaggcgtctgtacaacccttatactatgactattacggtggggaggtgggggaaggtaggatttttgcaggtcagaacaggttgtatcagcccgaagaaatcatcttggtttccttcgtgcttgttttcttttgcagcagtatctagtccaggagctaccccaccaaactgaagagtaaactgagaatgctgagtgccaggcattcaccatgctgttttgatgtctgtttttgatagttgcacactggggctgccacggataagcccatggcatacactgggctggctctccctcctctatccctctcccaggtgtgggaaggtcactttcactatgcttgtgaactaaatgctggctaacaagtgtcaaaccattagagtgccctgtggttctttcagtggtaacagttccaggggccaggctgtgaaaacactccccatgggcagatgtggcccaggagatgatacgcagcctgggtggggggttgggaacaccaggcagacagggaacagtgagaggagcccgtgactagaaaggagctgattacttttataggtcatgtagtggtctgtaagccgtggcctgcctctggctacttcccagcaaggtaatctgcctgcaactgctcattggttattttcattcgattccaagccttacgatggccttttaaggacatctctgctatctccactttcctttcccacatcctgatgctcttctccaggtccgcatttaagatcttctcccggacgtaagtcatcacctgtggtgcccggaactcggccagctgcttccggagcctcttattcactgcctcggctttggcccggtcctcctctacttgtagtgtttctttttcaattttttcaagtagctcttttctcagcaagatctccttgtccagattgaggtatatttccattgccttgtgaagcttgcttttgtaggcattgagaacctgcagagtgtttccagatgacagctttagctgggtcagttcttgattccttgcttcaattgtctcaagaaattgagcgttctctatcttcaactgctgaaaatcaacatcgtgaagggcctcactcacctcttccttctgcctcaattgtaaaagcatttttttcctctgaactttgagagaaacatttttcaaacgtaatttctccttcatattatccctccggcggttcatgtcctcaatgtatttcatcactttctgagtggccaaaatactccctttcttcttggatatggcttttagaatatctttttcaaactcatgcacttctctcgaaacttcactccatcgaatttcagcctcctcaatgatcgcctcgtgatgctgcaggtcgcgttccgcatttgcccttgtgtgtcgtaagtcatccttcatgtccgcaacctctttttgtaccagctcaagtttttggtcggcagtcaggcctaccccacggtccatacctgtccgggatttggatctacgcctgcctcgaaactgagctcctccaccagcccgcacagctggataacaggcagctccagctccgacccttcatgggagtcggagaggacgctctcggactcatcatcagtcatcactctgccgaagcggcccctgccaatgccgtgtgcccaggagctccgggtgccggcggccac

SEQ ID NO: 18349 - RNA, 4169 nt, Homo sapiens
  source 1..4169: mol_type = other RNA
tgaagtaccagctactcgagaggctgaggtgggagaattgcttgaatcccagaggtggaggttgcagtgagccaagattgcaccactgcactccagccttggggacagagaaagaaagagagaaagagagacagagagagtgaccaagacagaccacacacccaggtctcggatggtaaggggctgaagcggctgctcttctgcctttctgctgctcgtggttcagtctgttcagattgtttcctgttgttaattgcggccccattccatgtctcagtccaaactgcgagagcaacatgtcattgcctgggccttccagccaggcaggccacacaggtcagaagtggctggctagcctggggatgaccacccccttctcggaccaagatgggccatgggaggggcaggaattcctttgagaggagacctaggggtgtggggtctgggcaggtaaggtaagtgatacctactagttgccttgttgcttttcccattttccccaacttttcagaaaaatgctggcctttatagcgacatcaggatgatggtagctaatattctattgagtgtttgctgtgtgccaggcactgtgctgtgctcagcacgtgttacaggcattaactgtgttcccaccttggctcagagaggatttggtcacttgccagggtcccatatctagctaatgatgccaagcttctactccgtcactttaagttagataaagtgtatgtggcagaattcccaagtcccagaggactgctccattgggagtagggaagacccagagcacggccagccaggctggtaagcagttgccaggtggcaggaagtggcttacactaagggttgaagcaaggcagagaagggaaaatgtgagcatttcaggacaaaacagaaacaaacaccaacatttcaggaatgagaagccagaagagagggaaggtttggccaaaggactggaaaggggcaagaaaatgaaatatgaaccaggaagctataggcaatcagcagaagtccacagctaatttgcataataaaaggaaaagtcatcttgttggaatttgtggtggtggctgcctagatttgaaattgtatcctataatttgccccatttccagtgagaaccagcgtaaaacatttctagaacaaacagtatattgcacaaggatagatttacaacaaaaactagtttttctaagacttgaagccttctgtcttttatcacagggggacccaggaagcccaatgatgtgccagctacagcagttcgatctgtgggttctgagaggagtcctgaacttcggtggtgagacgtgccctggcctgtttctgtacaccaaggtggaagactacagcaaatggatcacatccaaggctgagagggccggccctcccctgtcctcactccaccactgggaaaagttgatttctttctcccaccatggaccaaatgccaccatgacacagaagacatattctgattctgaactgggccatgttggatcatacttgcagggacaaagaaggaccatcacgcattcacgactaggaaacagctctagagatagtctagatgttagggagaaggatgtaaaggaatcaggcaggtctcctgaggcgtctgtacaacccttatactatgactattacggtggggaggtgggggaaggtaggatttttgcaggtcagaacaggttgtatcagcccgaagaaatcatcttggtttccttcgtgcttgttttcttttgcagcagtatctagtccaggagctaccccaccaaactgaagagtaaactgagaatgctgagtgccaggcattcaccatgctgttttgatgtctgtttttgatagttgcacactggggctgccacggataagcccatggcatacactgggctggctctccctcctctatccctctcccaggtgtgggaaggtcactttcactatgcttgtgaactaaatgctggctaacaagtgtcaaaccattagagtgccctgtggttctttcagtggtaacagttccaggggccaggctgtgaaaacactccccatgggcagatgtggcccaggagatgatacgcagcctgggtggggggttgggaacaccaggcagacagggaacagtgagaggagcccgtgactagaaaggagctgattacttttataggtcatgtagtggtctgtaagccgtggcctgcctctggctacttcccagcaaggtaatctgcctgcaactgctcattggttattttcattcgattccaagccttacgatggccttttaaggacatctctgctatctccactttcctttcccacatcctgatgctcttctccaggtccgcatttaagatcttctcccggacgtaagtcatcacctgtggtgcccggaactcggccagctgcttccggagcctcttattcactgcctcggctttggcccggtcctcctctacttgtagtgtttctttttcaattttttcaagtagctcttttctcagcaagatctccttgtccagattgaggtatatttccattgccttgtgaagcttgcttttgtaggcattgagaacctgcagagtgtttccagatgacagctttagctgggtcagttcttgattccttgcttcaattgtctcaagaaattgagcgttctctatcttcaactgctgaaaatcaacatcgtgaagggcctcactcacctcttccttctgcctcaattgtaaaagcatttttttcctctgaactttgagagaaacatttttcaaacgtaatttctccttcatattatccctccggcggttcatgtcctcaatgtatttcatcactttctgagtggccaaaatactccctttcttcttggatatggcttttagaatatctttttcaaactcatgcacttctctcgaaacttcactccatcgaatttcagcctcctcaatgatcgcctcgtgatgctgcaggtcgcgttccgcatttgcccttgtgtgtcgtaagtcatccttcatgtccgcaacctctttttgtaccagctcaagtttttggtcggcagtcaggcctaccccacggtccatacctgtccgggatttggatctacgcctgcctcgaaactgtgcataatctgctgctgatattttaatttctgataatcgtggaggtcgctgatccctgggctccagtttagcgtaatatttctcaaacatctcagtctcagttttgagagcagagtttacatagagttccggaggccagaagtctggaggcaaggtgtctgcacagccactctccctctgaaggctctaggaggaatcttttcttgcctcttcccagcttctggtggctcctggcaatcttgtcattccttagattgtagctacatcactccaatctctgcctccatctttgcatggacttcttccctgtggctttgtgtgtcccctcctcttcttataaggacaccagttgtaagatttatttttctagaatcatgcagtgcattctcctttgtgactggcttcgttcattcaacatcatgttaatgagagttatccactttgatgaaggttaattatagatcgttcacgcttgttgctgtacagtattccattttgtttatctgttccactgttgatgagtatctggggagttcccagtttggggctattgcagtaagcactgctatgatcactccagtgtgtgtgtgtgtatgtctttcagtgagcacacagacacgtctctgctaggtatacacttaggagtagaattgctaggtcataaaatgttccactttagtagctgctgccaaatagttgtccagggtgattataccaggcactcaccttgaagatgtgaaacgagaagcaggtgctggggagccgcggggcacagggggcaccctctaggccttcaggacgggtgctttgctcgcccctctggattggctcagagcgttgccttcctgccccatcttcccaagttaggagagaccaattaggttaggagctctgcagagtgaagggagccaagattatgtcgtggctttcatttagggaatgagttgtgacgtgatgtatagacacttccaagtgtttgcctggtggaagcggctgaatgacgtgtacagtgggcataggcttggttaacccccagtcctggcatttatgtgt

SEQ ID NO: 18350 - RNA, 3583 nt, Homo sapiens
  source 1..3583: mol_type = other RNA
tgaagtaccagctactcgagaggctgaggtgggagaattgcttgaatcccagaggtggaggttgcagtgagccaagattgcaccactgcactccagccttggggacagagaaagaaagagagaaagagagacagagagagtgaccaagacagaccacacacccaggtctcggatggtaaggggctgaagcggctgctcttctgcctttctgctgctcgtggttcagtctgttcagattgtttcctgttgttaattgcggccccattccatgtctcagtccaaactgcgagagcaacatgtcattgcctgggccttccagccaggcaggccacacaggtcagaagtggctggctagcctggggatgaccacccccttctcggaccaagatgggccatgggaggggcaggaattcctttgagaggagacctaggggtgtggggtctgggcaggtaaggtaagtgatacctactagttgccttgttgcttttcccattttccccaacttttcagaaaaatgctggcctttatagcgacatcaggatgatggtagctaatattctattgagtgtttgctgtgtgccaggcactgtgctgtgctcagcacgtgttacaggcattaactgtgttcccaccttggctcagagaggatttggtcacttgccagggtcccatatctagctaatgatgccaagcttctactccgtcactttaagttagataaagtgtatgtggcagaattcccaagtcccagaggactgctccattgggagtagggaagacccagagcacggccagccaggctggtaagcagttgccaggtggcaggaagtggcttacactaagggttgaagcaaggcagagaagggaaaatgtgagcatttcaggacaaaacagaaacaaacaccaacatttcaggaatgagaagccagaagagagggaaggtttggccaaaggactggaaaggggcaagaaaatgaaatatgaaccaggaagctataggcaatcagcagaagtccacagctaatttgcataataaaaggaaaagtcatcttgttggaatttgtggtggtggctgcctagatttgaaattgtatcctataatttgccccatttccagtgagaaccagcgtaaaacatttctagaacaaacagtatattgcacaaggatagatttacaacaaaaactagtttttctaagacttgaagccttctgtcttttatcacagggggacccaggaagcccaatgatgtgccagctacagcagttcgatctgtgggttctgagaggagtcctgaacttcggtggtgagacgtgccctggcctgtttctgtacaccaaggtggaagactacagcaaatggatcacatccaaggctgagagggccggccctcccctgtcctcactccaccactgggaaaagttgatttctttctcccaccatggaccaaatgccaccatgacacagaagacatattctgattctgaactgggccatgttggatcatacttgcagggacaaagaaggaccatcacgcattcacgactaggaaacagctctagagatagtctagatgttagggagaaggatgtaaaggaatcaggcaggtctcctgaggcgtctgtacaacccttatactatgactattacggtggggaggtgggggaaggtaggatttttgcaggtcagaacaggttgtatcagcccgaagaaatcatcttggtttccttcgtgcttgttttcttttgcagcagtatctagtccaggagctaccccaccaaactgaagagtaaactgagaatgctgagtgccaggcattcaccatgctgttttgatgtctgtttttgatagttgcacactggggctgccacggataagcccatggcatacactgggctggctctccctcctctatccctctcccaggtgtgggaaggtcactttcactatgcttgtgaactaaatgctggctaacaagtgtcaaaccattagagtgccctgtggttctttcagtggtaacagttccaggggccaggctgtgaaaacactccccatgggcagatgtggcccaggagatgatacgcagcctgggtggggggttgggaacaccaggcagacagggaacagtgagaggagcccgtgactagaaaggagctgattacttttataggtcatgtagtggtctgtaagccgtggcctgcctctggctacttcccagcaaggtaatctgcctgcaactgctcattggttattttcattcgattccaagccttacgatggccttttaaggacatctctgctatctccactttcctttcccacatcctgatgctcttctccaggtccgcatttaagatcttctcccggacgtaagtcatcacctgtggtgcccggaactcggccagctgcttccggagcctcttattcactgcctcggctttggcccggtcctcctctacttgtagtgtttctttttcaattttttcaagtagctcttttctcagcaagatctccttgtccagattgaggtatatttccattgccttgtgaagcttgcttttgtaggcattgagaacctgcagagtgtttccagatgacagctttagctgggtcagttcttgattccttgcttcaattgtctcaagaaattgagcgttctctatcttcaactgctgaaaatcaacatcgtgaagggcctcactcacctcttccttctgcctcaattgtaaaagcatttttttcctctgaactttgagagaaacatttttcaaacgtaatttctccttcatattatccctccggcggttcatgtcctcaatgtatttcatcactttctgagtggccaaaatactccctttcttcttggatatggcttttagaatatctttttcaaactcatgcacttctctcgaaacttcactccatcgaatttcagcctcctcaatgatcgcctcgtgatgctgcaggtcgcgttccgcatttgcccttgtgtgtcgtaagtcatccttcatgtccgcaacctctttttgtaccagctcaagtttttggtcggcagtcaggcctaccccacggtccatacctgtccgggatttggatctacgcctgcctcgaaactgtgcataatctgctgctgatattttaatttctgataatcgtggaggtcgctgatccctgggctccagtttagcgtaatatttctcaaacatctcagtctcagttttgagagcagagtttacatagagttccggaggccagaagtctggaggcaaggtgtctgcacagccactctccctctgaaggctctaggaggaatcttttcttgcctcttcccagcttctggtggctcctggcaatcttgtcattccttagattgtagctacatcactccaatctctgcctccatctttgcatggacttcttccctgtggctttgtgtgtcccctcctcttcttataaggacaccagttgtaagatttatttttctggcctcttctttcccaaatgggaagctgctcaaaaatcagataaagggaccgggtgcagtggctcatgcctgtaattccagcactttgggaagccaagg

SEQ ID NO: 18351 - RNA, 3275 nt, Homo sapiens
  source 1..3275: mol_type = other RNA
tgaagtaccagctactcgagaggctgaggtgggagaattgcttgaatcccagaggtggaggttgcagtgagccaagattgcaccactgcactccagccttggggacagagaaagaaagagagaaagagagacagagagagtgaccaagacagaccacacacccaggtctcggatggtaaggggctgaagcggctgctcttctgcctttctgctgctcgtggttcagtctgttcagattgtttcctgttgttaattgcggccccattccatgtctcagtccaaactgcgagagcaacatgtcattgcctgggccttccagccaggcaggccacacaggtcagaagtggctggctagcctggggatgaccacccccttctcggaccaagatgggccatgggaggggcaggaattcctttgagaggagacctaggggtgtggggtctgggcaggtaaggtaagtgatacctactagttgccttgttgcttttcccattttccccaacttttcagaaaaatgctggcctttatagcgacatcaggatgatggtagctaatattctattgagtgtttgctgtgtgccaggcactgtgctgtgctcagcacgtgttacaggcattaactgtgttcccaccttggctcagagaggatttggtcacttgccagggtcccatatctagctaatgatgccaagcttctactccgtcactttaagttagataaagtgtatgtggcagaattcccaagtcccagaggactgctccattgggagtagggaagacccagagcacggccagccaggctggtaagcagttgccaggtggcaggaagtggcttacactaagggttgaagcaaggcagagaagggaaaatgtgagcatttcaggacaaaacagaaacaaacaccaacatttcaggaatgagaagccagaagagagggaaggtttggccaaaggactggaaaggggcaagaaaatgaaatatgaaccaggaagctataggcaatcagcagaagtccacagctaatttgcataataaaaggaaaagtcatcttgttggaatttgtggtggtggctgcctagatttgaaattgtatcctataatttgccccatttccagtgagaaccagcgtaaaacatttctagaacaaacagtatattgcacaaggatagatttacaacaaaaactagtttttctaagacttgaagccttctgtcttttatcacagggggacccaggaagcccaatgatgtgccagctacagcagttcgatctgtgggttctgagaggagtcctgaacttcggtggtgagacgtgccctggcctgtttctgtacaccaaggtggaagactacagcaaatggatcacatccaaggctgagagggccggccctcccctgtcctcactccaccactgggaaaagttgatttctttctcccaccatggaccaaatgccaccatgacacagaagacatattctgattctgaactgggccatgttggatcatacttgcagggacaaagaaggaccatcacgcattcacgactaggaaacagctctagagatagtctagatgttagggagaaggatgtaaaggaatcaggcaggtctcctgaggcgtctgtacaacccttatactatgactattacggtggggaggtgggggaaggtaggatttttgcaggtcagaacaggttgtatcagcccgaagaaatcatcttggtttccttcgtgcttgttttcttttgcagcagtatctagtccaggagctaccccaccaaactgaagagtaaactgagaatgctgagtgccaggcattcaccatgctgttttgatgtctgtttttgatagttgcacactggggctgccacggataagcccatggcatacactgggctggctctccctcctctatccctctcccaggtgtgggaaggtcactttcactatgcttgtgaactaaatgctggctaacaagtgtcaaaccattagagtgccctgtggttctttcagtggtaacagttccaggggccaggctgtgaaaacactccccatgggcagatgtggcccaggagatgatacgcagcctgggtggggggttgggaacaccaggcagacagggaacagtgagaggagcccgtgactagaaaggagctgattacttttataggtcatgtagtggtctgtaagccgtggcctgcctctggctacttcccagcaaggtaatctgcctgcaactgctcattggttattttcattcgattccaagccttacgatggccttttaaggacatctctgctatctccactttcctttcccacatcctgatgctcttctccaggtccgcatttaagatcttctcccggacgtaagtcatcacctgtggtgcccggaactcggccagctgcttccggagcctcttattcactgcctcggctttggcccggtcctcctctacttgtagtgtttctttttcaattttttcaagtagctcttttctcagcaagatctccttgtccagattgaggtatatttccattgccttgtgaagcttgcttttgtaggcattgagaacctgcagagtgtttccagatgacagctttagctgggtcagttcttgattccttgcttcaattgtctcaagaaattgagcgttctctatcttcaactgctgaaaatcaacatcgtgaagggcctcactcacctcttccttctgcctcaattgtaaaagcatttttttcctctgaactttgagagaaacatttttcaaacgtaatttctccttcatattatccctccggcggttcatgtcctcaatgtatttcatcactttctgagtggccaaaatactccctttcttcttggatatggcttttagaatatctttttcaaactcatgcacttctctcgaaacttcactccatcgaatttcagcctcctcaatgatcgcctcgtgatgctgcaggtcgcgttccgcatttgcccttgtgtgtcgtaagtcatccttcatgtccgcaacctctttttgtaccagctcaagtttttggtcggcagtcaggcctaccccacggtccatacctgtccgggatttggatctacgcctgcctcgaaactgtgcataatctgctgctgatattttaatttctgataatcgtggaggtcgctgatccctgggctccagtttagcgtaatatttctcaaacatctcagtctcagttttgagagcagagtttacatagctccacctcctgtagtgcattcaccacacaacagc

SEQ ID NO: 18352 - RNA, 3420 nt, Homo sapiens
  source 1..3420: mol_type = other RNA
tgaagtaccagctactcgagaggctgaggtgggagaattgcttgaatcccagaggtggaggttgcagtgagccaagattgcaccactgcactccagccttggggacagagaaagaaagagagaaagagagacagagagagtgaccaagacagaccacacacccaggtctcggatggtaaggggctgaagcggctgctcttctgcctttctgctgctcgtggttcagtctgttcagattgtttcctgttgttaattgcggccccattccatgtctcagtccaaactgcgagagcaacatgtcattgcctgggccttccagccaggcaggccacacaggtcagaagtggctggctagcctggggatgaccacccccttctcggaccaagatgggccatgggaggggcaggaattcctttgagaggagacctaggggtgtggggtctgggcaggtaaggtaagtgatacctactagttgccttgttgcttttcccattttccccaacttttcagaaaaatgctggcctttatagcgacatcaggatgatggtagctaatattctattgagtgtttgctgtgtgccaggcactgtgctgtgctcagcacgtgttacaggcattaactgtgttcccaccttggctcagagaggatttggtcacttgccagggtcccatatctagctaatgatgccaagcttctactccgtcactttaagttagataaagtgtatgtggcagaattcccaagtcccagaggactgctccattgggagtagggaagacccagagcacggccagccaggctggtaagcagttgccaggtggcaggaagtggcttacactaagggttgaagcaaggcagagaagggaaaatgtgagcatttcaggacaaaacagaaacaaacaccaacatttcaggaatgagaagccagaagagagggaaggtttggccaaaggactggaaaggggcaagaaaatgaaatatgaaccaggaagctataggcaatcagcagaagtccacagctaatttgcataataaaaggaaaagtcatcttgttggaatttgtggtggtggctgcctagatttgaaattgtatcctataatttgccccatttccagtgagaaccagcgtaaaacatttctagaacaaacagtatattgcacaaggatagatttacaacaaaaactagtttttctaagacttgaagccttctgtcttttatcacagggggacccaggaagcccaatgatgtgccagctacagcagttcgatctgtgggttctgagaggagtcctgaacttcggtggtgagacgtgccctggcctgtttctgtacaccaaggtggaagactacagcaaatggatcacatccaaggctgagagggccggccctcccctgtcctcactccaccactgggaaaagttgatttctttctcccaccatggaccaaatgccaccatgacacagaagacatattctgattctgaactgggccatgttggatcatacttgcagggacaaagaaggaccatcacgcattcacgactaggaaacagctctagagatagtctagatgttagggagaaggatgtaaaggaatcaggcaggtctcctgaggcgtctgtacaacccttatactatgactattacggtggggaggtgggggaaggtaggatttttgcaggtcagaacaggttgtatcagcccgaagaaatcatcttggtttccttcgtgcttgttttcttttgcagcagtatctagtccaggagctaccccaccaaactgaagagtaaactgagaatgctgagtgccaggcattcaccatgctgttttgatgtctgtttttgatagttgcacactggggctgccacggataagcccatggcatacactgggctggctctccctcctctatccctctcccaggtgtgggaaggtcactttcactatgcttgtgaactaaatgctggctaacaagtgtcaaaccattagagtgccctgtggttctttcagtggtaacagttccaggggccaggctgtgaaaacactccccatgggcagatgtggcccaggagatgatacgcagcctgggtggggggttgggaacaccaggcagacagggaacagtgagaggagcccgtgactagaaaggagctgattacttttataggtcatgtagtggtctgtaagccgtggcctgcctctggctacttcccagcaaggtaatctgcctgcaactgctcattggttattttcattcgattccaagccttacgatggccttttaaggacatctctgctatctccactttcctttcccacatcctgatgctcttctccaggtccgcatttaagatcttctcccggacgtaagtcatcacctgtggtgcccggaactcggccagctgcttccggagcctcttattcactgcctcggctttggcccggtcctcctctacttgtagtgtttctttttcaattttttcaagtagctcttttctcagcaagatctccttgtccagattgaggtatatttccattgccttgtgaagcttgcttttgtaggcattgagaacctgcagagtgtttccagatgacagctttagctgggtcagttcttgattccttgcttcaattgtctcaagaaattgagcgttctctatcttcaactgctgaaaatcaacatcgtgaagggcctcactcacctcttccttctgcctcaattgtaaaagcatttttttcctctgaactttgagagaaacatttttcaaacgtaatttctccttcatattatccctccggcggttcatgtcctcaatgtatttcatcactttctgagtggccaaaatactccctttcttcttggatatggcttttagaatatctttttcaaactcatgcacttctctcgaaacttcactccatcgaatttcagcctcctcaatgatcgcctcgtgatgctgcaggtcgcgttccgcatttgcccttgtgtgtcgtaagtcatccttcatgtccgcaacctctttttgtaccagctcaagtttttggtcggcagtcaggcctaccccacggtccatacctgtccgggatttggatctacgcctgcctcgaaactgtgcataatctgctgctgatattttaatttctgataatcgtggaggtcgctgatccctgggctccagtttagcgtaatatttctcaaacatctcagtctcagttttgagagcagagtttacatagctgagctcctccaccagcccgcacagctggataacaggcagctccagctccgacccttcatgggagtcggagaggacgctctcggactcatcatcagtcatcactctgccgaagcggcccctgccaatgccgtgtgcccaggagctccgggtgccggcggccacgcgtcactccggctgc

SEQ ID NO: 18353 - RNA, 3261 nt, Homo sapiens
  source 1..3261: mol_type = other RNA
tgaagtaccagctactcgagaggctgaggtgggagaattgcttgaatcccagaggtggaggttgcagtgagccaagattgcaccactgcactccagccttggggacagagaaagaaagagagaaagagagacagagagagtgaccaagacagaccacacacccaggtctcggatggtaaggggctgaagcggctgctcttctgcctttctgctgctcgtggttcagtctgttcagattgtttcctgttgttaattgcggccccattccatgtctcagtccaaactgcgagagcaacatgtcattgcctgggccttccagccaggcaggccacacaggtcagaagtggctggctagcctggggatgaccacccccttctcggaccaagatgggccatgggaggggcaggaattcctttgagaggagacctaggggtgtggggtctgggcaggtaaggtaagtgatacctactagttgccttgttgcttttcccattttccccaacttttcagaaaaatgctggcctttatagcgacatcaggatgatggtagctaatattctattgagtgtttgctgtgtgccaggcactgtgctgtgctcagcacgtgttacaggcattaactgtgttcccaccttggctcagagaggatttggtcacttgccagggtcccatatctagctaatgatgccaagcttctactccgtcactttaagttagataaagtgtatgtggcagaattcccaagtcccagaggactgctccattgggagtagggaagacccagagcacggccagccaggctggtaagcagttgccaggtggcaggaagtggcttacactaagggttgaagcaaggcagagaagggaaaatgtgagcatttcaggacaaaacagaaacaaacaccaacatttcaggaatgagaagccagaagagagggaaggtttggccaaaggactggaaaggggcaagaaaatgaaatatgaaccaggaagctataggcaatcagcagaagtccacagctaatttgcataataaaaggaaaagtcatcttgttggaatttgtggtggtggctgcctagatttgaaattgtatcctataatttgccccatttccagtgagaaccagcgtaaaacatttctagaacaaacagtatattgcacaaggatagatttacaacaaaaactagtttttctaagacttgaagccttctgtcttttatcacagggggacccaggaagcccaatgatgtgccagctacagcagttcgatctgtgggttctgagaggagtcctgaacttcggtggtgagacgtgccctggcctgtttctgtacaccaaggtggaagactacagcaaatggatcacatccaaggctgagagggccggccctcccctgtcctcactccaccactgggaaaagttgatttctttctcccaccatggaccaaatgccaccatgacacagaagacatattctgattctgaactgggccatgttggatcatacttgcagggacaaagaaggaccatcacgcattcacgactaggaaacagctctagagatagtctagatgttagggagaaggatgtaaaggaatcaggcaggtctcctgaggcgtctgtacaacccttatactatgactattacggtggggaggtgggggaaggtaggatttttgcaggtcagaacaggttgtatcagcccgaagaaatcatcttggtttccttcgtgcttgttttcttttgcagcagtatctagtccaggagctaccccaccaaactgaagagtaaactgagaatgctgagtgccaggcattcaccatgctgttttgatgtctgtttttgatagttgcacactggggctgccacggataagcccatggcatacactgggctggctctccctcctctatccctctcccaggtgtgggaaggtcactttcactatgcttgtgaactaaatgctggctaacaagtgtcaaaccattagagtgccctgtggttctttcagtggtaacagttccaggggccaggctgtgaaaacactccccatgggcagatgtggcccaggagatgatacgcagcctgggtggggggttgggaacaccaggcagacagggaacagtgagaggagcccgtgactagaaaggagctgattacttttataggtcatgtagtggtctgtaagccgtggcctgcctctggctacttcccagcaaggtaatctgcctgcaactgctcattggttattttcattcgattccaagccttacgatggccttttaaggacatctctgctatctccactttcctttcccacatcctgatgctcttctccaggtccgcatttaagatcttctcccggacgtaagtcatcacctgtggtgcccggaactcggccagctgcttccggagcctcttattcactgcctcggctttggcccggtcctcctctacttgtagtgtttctttttcaattttttcaagtagctcttttctcagcaagatctccttgtccagattgaggtatatttccattgccttgtgaagcttgcttttgtaggcattgagaacctgcagagtgtttccagatgacagctttagctgggtcagttcttgattccttgcttcaattgtctcaagaaattgagcgttctctatcttcaactgctgaaaatcaacatcgtgaagggcctcactcacctcttccttctgcctcaattgtaaaagcatttttttcctctgaactttgagagaaacatttttcaaacgtaatttctccttcatattatccctccggcggttcatgtcctcaatgtatttcatcactttctgagtggccaaaatactccctttcttcttggatatggcttttagaatatctttttcaaactcatgcacttctctcgaaacttcactccatcgaatttcagcctcctcaatgatcgcctcgtgatgctgcaggtcgcgttccgcatttgcccttgtgtgtcgtaagtcatccttcatgtccgcaacctctttttgtaccagctcaagtttttggtcggcagtcaggcctaccccacggtccatacctgtccgggatttggatctacgcctgcctcgaaactgtgcataatctgctgctgatattttaatttctgataatcgtggaggtcgctgatccctgggctccagtttagcgtaatatttctcaaacatctcagtctcagttttgagagcagagtttacatagctggcctaattggcatcatgg

SEQ ID NO: 18354 - RNA, 3693 nt, Homo sapiens
  source 1..3693: mol_type = other RNA
tgaagtaccagctactcgagaggctgaggtgggagaattgcttgaatcccagaggtggaggttgcagtgagccaagattgcaccactgcactccagccttggggacagagaaagaaagagagaaagagagacagagagagtgaccaagacagaccacacacccaggtctcggatggtaaggggctgaagcggctgctcttctgcctttctgctgctcgtggttcagtctgttcagattgtttcctgttgttaattgcggccccattccatgtctcagtccaaactgcgagagcaacatgtcattgcctgggccttccagccaggcaggccacacaggtcagaagtggctggctagcctggggatgaccacccccttctcggaccaagatgggccatgggaggggcaggaattcctttgagaggagacctaggggtgtggggtctgggcaggtaaggtaagtgatacctactagttgccttgttgcttttcccattttccccaacttttcagaaaaatgctggcctttatagcgacatcaggatgatggtagctaatattctattgagtgtttgctgtgtgccaggcactgtgctgtgctcagcacgtgttacaggcattaactgtgttcccaccttggctcagagaggatttggtcacttgccagggtcccatatctagctaatgatgccaagcttctactccgtcactttaagttagataaagtgtatgtggcagaattcccaagtcccagaggactgctccattgggagtagggaagacccagagcacggccagccaggctggtaagcagttgccaggtggcaggaagtggcttacactaagggttgaagcaaggcagagaagggaaaatgtgagcatttcaggacaaaacagaaacaaacaccaacatttcaggaatgagaagccagaagagagggaaggtttggccaaaggactggaaaggggcaagaaaatgaaatatgaaccaggaagctataggcaatcagcagaagtccacagctaatttgcataataaaaggaaaagtcatcttgttggaatttgtggtggtggctgcctagatttgaaattgtatcctataatttgccccatttccagtgagaaccagcgtaaaacatttctagaacaaacagtatattgcacaaggatagatttacaacaaaaactagtttttctaagacttgaagccttctgtcttttatcacagggggacccaggaagcccaatgatgtgccagctacagcagttcgatctgtgggttctgagaggagtcctgaacttcggtggtgagacgtgccctggcctgtttctgtacaccaaggtggaagactacagcaaatggatcacatccaaggctgagagggccggccctcccctgtcctcactccaccactgggaaaagttgatttctttctcccaccatggaccaaatgccaccatgacacagaagacatattctgattctgaactgggccatgttggatcatacttgcagggacaaagaaggaccatcacgcattcacgactaggaaacagctctagagatagtctagatgttagggagaaggatgtaaaggaatcaggcaggtctcctgaggcgtctgtacaacccttatactatgactattacggtggggaggtgggggaaggtaggatttttgcaggtcagaacaggttgtatcagcccgaagaaatcatcttggtttccttcgtgcttgttttcttttgcagcagtatctagtccaggagctaccccaccaaactgaagagtaaactgagaatgctgagtgccaggcattcaccatgctgttttgatgtctgtttttgatagttgcacactggggctgccacggataagcccatggcatacactgggctggctctccctcctctatccctctcccaggtgtgggaaggtcactttcactatgcttgtgaactaaatgctggctaacaagtgtcaaaccattagagtgccctgtggttctttcagtggtaacagttccaggggccaggctgtgaaaacactccccatgggcagatgtggcccaggagatgatacgcagcctgggtggggggttgggaacaccaggcagacagggaacagtgagaggagcccgtgactagaaaggagctgattacttttataggtcatgtagtggtctgtaagccgtggcctgcctctggctacttcccagcaaggtaatctgcctgcaactgctcattggttattttcattcgattccaagccttacgatggccttttaaggacatctctgctatctccactttcctttcccacatcctgatgctcttctccaggtccgcatttaagatcttctcccggacgtaagtcatcacctgtggtgcccggaactcggccagctgcttccggagcctcttattcactgcctcggctttggcccggtcctcctctacttgtagtgtttctttttcaattttttcaagtagctcttttctcagcaagatctccttgtccagattgaggtatatttccattgccttgtgaagcttgcttttgtaggcattgagaacctgcagagtgtttccagatgacagctttagctgggtcagttcttgattccttgcttcaattgtctcaagaaattgagcgttctctatcttcaactgctgaaaatcaacatcgtgaagggcctcactcacctcttccttctgcctcaattgtaaaagcatttttttcctctgaactttgagagaaacatttttcaaacgtaatttctccttcatattatccctccggcggttcatgtcctcaatgtatttcatcactttctgagtggccaaaatactccctttcttcttggatatggcttttagaatatctttttcaaactcatgcacttctctcgaaacttcactccatcgaatttcagcctcctcaatgatcgcctcgtgatgctgcaggtcgcgttccgcatttgcccttgtgtgtcgtaagtcatccttcatgtccgcaacctctttttgtaccagctcaagtttttggtcggcagtcaggcctaccccacggtccatacctgtccgggatttggatctacgcctgcctcgaaactgtgcataatctgctgctgatattttaatttctgataatcgtggaggtcgctgatccctgggctccagtttagcgtaatatttctcaaacatctcagtctcagttttgagagcagagtttacatagctggtccaaattgctgctgtagaattgtggatcggctaagcacaccgtctggcatgagagagactcctccggctgaaaccctcacttccccaattaccctctgggcttctcaccaccggccccatcccctcgccctaccaccccgttctagctccaccaacagcttgttggctcagtggtggtggagtaaggagtaaagaggaaaagtctccccagtgctcagtgagggcttggatcttctccatgctggtccccaagtccgaggccgcccggagaggagggcctaggaggaagaggggcggcccccaggcgcgggcggcggtacctgagctcctccaccagcccgcacagctggataacaggcagctccagctccgacccttcatgggagtcggagaggacgctctcggactcatcatcagtcatcactctgccgaagcggcccctgccaat

SEQ ID NO: 18355 - RNA, 3258 nt, Homo sapiens
  source 1..3258: mol_type = other RNA
tgaagtaccagctactcgagaggctgaggtgggagaattgcttgaatcccagaggtggaggttgcagtgagccaagattgcaccactgcactccagccttggggacagagaaagaaagagagaaagagagacagagagagtgaccaagacagaccacacacccaggtctcggatggtaaggggctgaagcggctgctcttctgcctttctgctgctcgtggttcagtctgttcagattgtttcctgttgttaattgcggccccattccatgtctcagtccaaactgcgagagcaacatgtcattgcctgggccttccagccaggcaggccacacaggtcagaagtggctggctagcctggggatgaccacccccttctcggaccaagatgggccatgggaggggcaggaattcctttgagaggagacctaggggtgtggggtctgggcaggtaaggtaagtgatacctactagttgccttgttgcttttcccattttccccaacttttcagaaaaatgctggcctttatagcgacatcaggatgatggtagctaatattctattgagtgtttgctgtgtgccaggcactgtgctgtgctcagcacgtgttacaggcattaactgtgttcccaccttggctcagagaggatttggtcacttgccagggtcccatatctagctaatgatgccaagcttctactccgtcactttaagttagataaagtgtatgtggcagaattcccaagtcccagaggactgctccattgggagtagggaagacccagagcacggccagccaggctggtaagcagttgccaggtggcaggaagtggcttacactaagggttgaagcaaggcagagaagggaaaatgtgagcatttcaggacaaaacagaaacaaacaccaacatttcaggaatgagaagccagaagagagggaaggtttggccaaaggactggaaaggggcaagaaaatgaaatatgaaccaggaagctataggcaatcagcagaagtccacagctaatttgcataataaaaggaaaagtcatcttgttggaatttgtggtggtggctgcctagatttgaaattgtatcctataatttgccccatttccagtgagaaccagcgtaaaacatttctagaacaaacagtatattgcacaaggatagatttacaacaaaaactagtttttctaagacttgaagccttctgtcttttatcacagggggacccaggaagcccaatgatgtgccagctacagcagttcgatctgtgggttctgagaggagtcctgaacttcggtggtgagacgtgccctggcctgtttctgtacaccaaggtggaagactacagcaaatggatcacatccaaggctgagagggccggccctcccctgtcctcactccaccactgggaaaagttgatttctttctcccaccatggaccaaatgccaccatgacacagaagacatattctgattctgaactgggccatgttggatcatacttgcagggacaaagaaggaccatcacgcattcacgactaggaaacagctctagagatagtctagatgttagggagaaggatgtaaaggaatcaggcaggtctcctgaggcgtctgtacaacccttatactatgactattacggtggggaggtgggggaaggtaggatttttgcaggtcagaacaggttgtatcagcccgaagaaatcatcttggtttccttcgtgcttgttttcttttgcagcagtatctagtccaggagctaccccaccaaactgaagagtaaactgagaatgctgagtgccaggcattcaccatgctgttttgatgtctgtttttgatagttgcacactggggctgccacggataagcccatggcatacactgggctggctctccctcctctatccctctcccaggtgtgggaaggtcactttcactatgcttgtgaactaaatgctggctaacaagtgtcaaaccattagagtgccctgtggttctttcagtggtaacagttccaggggccaggctgtgaaaacactccccatgggcagatgtggcccaggagatgatacgcagcctgggtggggggttgggaacaccaggcagacagggaacagtgagaggagcccgtgactagaaaggagctgattacttttataggtcatgtagtggtctgtaagccgtggcctgcctctggctacttcccagcaaggtaatctgcctgcaactgctcattggttattttcattcgattccaagccttacgatggccttttaaggacatctctgctatctccactttcctttcccacatcctgatgctcttctccaggtccgcatttaagatcttctcccggacgtaagtcatcacctgtggtgcccggaactcggccagctgcttccggagcctcttattcactgcctcggctttggcccggtcctcctctacttgtagtgtttctttttcaattttttcaagtagctcttttctcagcaagatctccttgtccagattgaggtatatttccattgccttgtgaagcttgcttttgtaggcattgagaacctgcagagtgtttccagatgacagctttagctgggtcagttcttgattccttgcttcaattgtctcaagaaattgagcgttctctatcttcaactgctgaaaatcaacatcgtgaagggcctcactcacctcttccttctgcctcaattgtaaaagcatttttttcctctgaactttgagagaaacatttttcaaacgtaatttctccttcatattatccctccggcggttcatgtcctcaatgtatttcatcactttctgagtggccaaaatactccctttcttcttggatatggcttttagaatatctttttcaaactcatgcacttctctcgaaacttcactccatcgaatttcagcctcctcaatgatcgcctgtgcataatctgctgctgatattttaatttctgataatcgtggaggtcgctgatccctgggctccagtttagcgtaatatttctcaaacatctcagtctcagttttgagagcagagtttacatagctgagctcctccaccagcccgcacagctggataacaggcagctccagctccgacccttcatgggagtcggagaggacgctctcggactcatcatcagtcatcactctgccgaagcggcccctgccaatgccgtgtgcccaggagctccgggtgccggcggccacgcgtcactccggctgc

SEQ ID NO: 18356 - RNA, 1636 nt, Homo sapiens
  source 1..1636: mol_type = other RNA
tgaagtaccagctactcgagaggctgaggtgggaggatcccttggatccaggagttcaaggccacaataagtggttatcacaacactgcactccagcctgggtgacagcgtgaggctctctctcaaaaaaaaaaaaaaaaaaaaaaacaaactaaaagttacagttcatgtctcacgttcacaaaggtcttcccaccggctaactgctaagtctaagaaacagcctggggttacagaatgtgaaatgcagtatacattcgtaattccttatccagaatgctgaaatccacaacattatgaaaactgggttttccttaagctcgatgtcaaaattcaatgagcggcaaaatctgacctaaactgagtcatggctatttataatcttaactcctcccccttactgtgaatactcacatttcactggagagctgtgtgaatgtgcctgattacagggtgcagtcctagaccccacctggggattacataatacacctcttatacattgtactatcttcctaaaatctgaaaaattctgaactctgaaacacatacagccccaaccattccagagaaagcactgtggacctatgtaacatgccctggtccaagaagaaactcacttgccatttgaagaaacaaagcatacagcacaggaaaagatatcctgtgatacaaggtaagaaacctgcctgatgacagggctgacggaaggaagaaagaaaggggacaaaatggttttaggtgcaaggatttggagaagaccactgtatgaagacagcccgctgtgtggccagagtgacgccatcctgaagcaaaaccaccgtgatgaccgatgctcgactcgtgcatgccaagctgttctgcaatgaggtctgaagacgatgcctccggcacaggcaacctctcatcaagatgctcatccagcctgaccagtggtcccaagtgttgtcaagcaagtcagaagacagggccggctgcacacgttctaccctgaaagcttatctccagctggcgctggatgcggcctttgctccgctcccgaaacagagtctgtgcctcattgtactccgccatggcttccacaaacttccgagacagcaccgaatgctgggttcttcgtatccgaagatccactgaagtccggttcccactctcatcctgatcaaaactttgttcaatagcctttaacttggctcgaattttattcgcagttttcttgatttctttgttcagatcttcaagctcttcttttatttttccttccgggtttggtgcagaaagaatgatgctgtggtttttctttacttcttcaacatattgagttattttatcaatactgtttctaatctcctccacctgatggaagaaatcatccatgaaatgatctttctcaaccacaacaactgtgtctccatcatcattcttcctacacgccgtcaggtctggcagccggtcccgcatccccgccggccgggcagcgcgccccgccgctcaagcctgtcccgagctgcctccggccgggcctcgggctctccggtctccgcctcaggccccgcggtcccggcccggcgccagcagccctccctggagccggcgctgccacggcaaccgcgccccgcgcgctctgcgcatgccc

SEQ ID NO: 18357 - RNA, 250 nt, Homo sapiens
  source 1..250: mol_type = other RNA
tgaagtaccagctactcgagaggctgaggtgggaggatctcttgagccctggaagcggaggttgcggtgagccataatcacgccgctgcactccagcctgggcaacagagcaagaccctgtcttaaaaaaacaaatagagccaggcacagtggctcatacttgtaatcccagcactttgggaggccaaggcaggcagatcacctgaggtcaggagttcgagaccagcctggccaacatatagtgaaactc

SEQ ID NO: 18358 - RNA, 6343 nt, Homo sapiens
  source 1..6343: mol_type = other RNA
tgaagtaccagctactcgagaggctgattgcagcagtacactccaacctgggcaaatgaagtaagaccctgtctcagaaaaaaaaaaaaaaaaaaaaatttctacatggaatggtcatcctcatcctcacttgaaatactcttgtaacaggtggttccagtgttttaaacccattaagaggacttccacagctaaactttctatggactggccacttgtatttctacctgtatttccaggtatctcaattccttgaatgtagcctcaattgttctgttctgggacctttgcctgtatttcctcctgttcctccacctgaactgctcaccgttcagaggttcttcctctcacttcacaaattcctacagattctcaaaatctcagctaaaagctcatacaaattttgagccttctggtagcaactattttacaacctcatgaaatttaccagagccgcaattgcctaatacattatgaatgataaaattatgaataagaccttcaactctggatatgagatctgtcgacttctggcactcacgtttaatcacacattcctagttccttctttttggctttaagtttaaaacatgtaagaaactggctgggcgtggtggctcatgcttgtaatcccagcacttttgagaggccagcactttgagaggctgaggtgggaggatcactggaggtcaggaggtcgagaccagcctggccaacatggtgaaaacccatctctactaaaagtacaaaaatcagctgggctcagtggcacacgcctgtaatcccgactacttggaatgctgaggcacgagaatcgcttgaacccgggagatgacagctgtagtgagccgagatcatgccactgcactccagcctgggcaacagagcaagactctatctcaaaaataaaaataaatggataaaacatgtaagaaactaaaaagcaatgcttttatgtaatattttatcctgggtttcaaaataataaaactcagtttgttctaggatccacaaaacttaaaatgcccaatttcccataggaaaattaaacaaccagactgacttatttcccgccagtaatctattatttctaaataccccatttcttcttttattcagactcttggcttgaggatgacatggtcgggcctcaataagcccactgtaagtcaaaaatatcataagtagaagatgtgtttaatactccaataaactcataaagctgaagtcttaagtcaaaccattataagtcagggactgtctgtactaagattttagtgaataacttaatttttgtaaactggaaaacctgacaatatgatgtcaaaaggaagaaacacaagatacaaagcatactgtatttttgaaaatatacatcaatcaaaatttcttatgaatacttatccttgagtaaaataatttcatataccaacaaggatgtttccatttctgtaaagtcatgtaagtgatcctcaatcagtccaagaacttggctttttatccaggttatattttaatatctggagttttaatccagcatacaaaaatcaccagtatacatctattaagttaactgcagtattatttcaccatcaccatttacatgtacttttcaggtatcagagacttagtgctttaagtagcaaattacctaaattatgaacacatatttccaaaaacaaaatcaagctcataattaccaagtatatatgtacagtgcagattaaaaaaaaactgaattagcacatatttctcttttctaaagctcctatgaagaacttacactcttctgcactaccaatctattctgtacatttaaaataacatttgttttgatttaaagtcaaaaatataaaggcttaaatttttgtaagactaacccataaaaaaggactccaattttaaaccaatccctgaaaccaaagcattcaaatatttgaatattagttcaatatttctacatagcacgataagattttcagttacttcaagttttgtctttatttttaataatgggaatggcctacaattacaataaacaattaattcagttattttaggggccttaccatatcattaacctattcacacaacaaaaatatttttatgaaagttaatatatcctttcctgattaagtgtgctaaaacagaaatagaggtagaatcccatttttcttaagtaccactctacaagccagttccacacaattaaggtatttttgcaatctaaaatagtgatgctaatactgcttcagtaagctagatttactaatttaagaatcctaagaaattatatatgtggctttcagacatccatgttaaactatcaacttgtggaatttgtggaacacttaccctacttgagtgaccataaagcaaacaactctaaaattttttcatatcagttttctttataagtgattatatgatatttcaccatttctaacaggaaaaaatgagacttacttggcagtgtgcatgggctgctggaaactacaatcagagtgtaaagacaaatctcaaaaatgtttgtagataactcagaataataacccagaatataacctatcaggaactatggaattccattttagtcttcaaataataaactccacttagcagggattgtgaggttgctcttaaaattatatatttacagaacatagtggcctcagcacaaaatagctccctctagacatcactactctccactcttcaaaaaaaaagtatatacattcatttaaaaaaaaacacccaaaatatcaccagtacattttataaaattaaatccaaattttattaaggatttcaggttacatacttcaaatttctagaatggaatggaatcattttggaactggaaaaatggcataaacactgacgtcccttaaaacttcaattttataaagaaaattcttctgcaaaccacatcccctttatgtaacaagactaggtattatctacaccttcactttggcaatagctatttcctaaagaatgaaaaagatgattttgctacttcagttcattaaaaatgggattctatctttgaagttcagaaaaagctgcatttcgatgaactatggttaaaaaaaaaaagcacatagtgtctaatcaaagcaaaggaaatcattttgaaaataaagaaaaaaagctattataattggttaaggatttccagtagtaagttaaaatctcaggagaggaatggatagcactacaaacaatgtgttcacattccaagaccttaacactaacttctcagaaaggaagttttcattacctctaaaaatcaattcaatgtaattttattaagagcaggaaatctagaccttcctctaatgacaatccaataatccaccctcactgtcaaaaaaaagttcaaccccaaaattaacagtaattagcctgaggtattgtaaatgtggctctacagtctgaaatttaatggcatcttttgtcaaaaatagtcttatttccactttaagtctcatgactacaatactatagtgctatccctgtagtatttacaatacagtcatcaaaaatatctgaaaacaaatcttggaccttgtgaaatagtgcatccctccacttctataaaaataggagccacacaaagatctaaaaagagtgctgactgcccagatccagaacagaggtacttaacacctttgttttccagtttagttatcaaagcgtggtgtgaacaaaatgcttagtgtcacactggcattacaaataggcccaaaattttgagcttttaacaagattgagaaacattatatgagatttaactcaatatgccttaacacatccatgaggtagttaggtaaacagtactacccattttaattacacagtaaacagaagcacgggtaagtgacatactcatactttaagcaataagaattagaagaaaccatagaagcttggggccttctctctagctctaacccaaagaaaatgaatttttttttttttttttaaaagaaaacagcatcaatcacttaagattttcttcctcttttttttttttttttacacttgcttattagtatagcatctcgttccaaagctggtaccttttcttcaacaatgtgttaaaaactgagtataacccttaattcaaggtaggcctctacttctacctgaattggtacaaaattaagacattatcttgtaagaactaaaattgtatttgaaatttttattttagctgcaaaaacaaaaacaagcaaacaaacaacaaataacttgaaaataggcttgtcaaatgatgtaaattcatcctttccagggaagcagaaggtagaccctaccacaaagaaaagatgcttagttaatggaggttaaatttaaaaatacagttaaattcaggctaacttctgaaaatcccgttttattcacctcactgtggtaccagtaactatactgagtcaggttactttacagttaactatgtcacctaaaacacaataatccattaacactctaataacagttattgggtgtggtcatactggaaattcttaaccatatagttgtcttgccaattttttttttaaacaataaattgtcttagtataagtcactgcatttctgtaacaaagtaatgaaaggcacagctaatccaagcggacttaaccctattcaacaaccagctgaaaaaatactttggttcttcaaggaaaaaattacaaaaaaaaaaaaaaggtatttcctttaacagttgttaattttcatagctgtactccaagagctacataaaaatattccagaagaaccaaattatgtagcaatgaatgaacatgcgtgacagaatttgtgcattcaacatagctggcagaaaaactagttaaaatgctaggtagaacaaattggtctttaaaatatcagtttcctgtcctttaaaaaaaaattacctagtctaccaagaaaatacaaaaacataaggctgtaagtaaataagagttgtgtttaggctattacagtgcaggttatcctcaaggccacatacatcctgcttcactgctgcttgcactctgctgggttttgatccttctttgggtcatagtctggatcattttcctcatctccttcttcttccccttcctcatccgcttcttcaccttcttcatcataatcatcatcatcatcttcaatagcttctccagtaaaatataacactgatcttgggattatacgctcacgtaaaaagtgaccaatttcgaagtctgcagcaaggatagcttcagcatcatcatccagatctccactctcaggaacttcaggaggggcaaaaaagttaaagaaagagtcattggaaactgttttagtcacagtacgaactgtcccacgtcccttgtgtttctgcttcttcttaatagttttcaaagtgacattctttccttttttccaatctatctggcaccctgtacaacccataatttctggtccatcaaaagaaaagggatcagaatcatctggttctgacctcatcctgtatgtctttgtcagcacttcatttgtaaaatattcattgggttcaaagtgaaattctaagacaaaactcataggctggccagcatctgagaacttcactttaatatctttcaagtgcttcagaataggttcatcgtgttcctgaaccatatcactgagcaagtcaacattcttaaaaacagttaaccaaaattcaggaattcctttggggtcttctttttcttcatcttttttctcatcttcaatcttggccttttctttcaattcctccgaaatctcatcttcttcatctggtttccattcacattcttcttccgtaggttcataaattgcattaataatttcaaatcgcttatcaaatagaggctgatagagaacagcatacttcctttcaagatcgtgaacttcctcatagaatttggcttctatctgtgcacatttaacttgcaggtttttgagagcattcactcgtcttttaactaccctaggcaggctttcaatgtatcctgttggtgtttctaccagaccatcaagtctttcttgaagggctgcaagaatctgaggattttgcatcatctgaacagttagctgacgtgctttgagttttgtttcttcaccagtttcctcttcttctacttcttcaacatcatccaaatcttgatcaagttcagactgttctttgttgtcaatgtctgccatgttgtaagaactccaaatatcggcgactagtatggggagccaggcggccggagctgcgcaggcagtgactcagggcggcagcggcagcagcagcgggaggagcaggaggcggcgccgcgagcagatggcgctaaaaaag

SEQ ID NO: 18359 - RNA, 3622 nt, Homo sapiens
  source 1..3622: mol_type = other RNA
tgaagtaccagctactcgagaggctgcagcttgagtccaggagttcaaggctgcagggagccataatcatgccactgcactccagcctgggagacagtgagaacttggctcttaaaaaaaaaaaggaaaaaaaattgataacgacaatttgtaatggtcagtcctatccaccagtctaaatgaaagtttaaaaattttcatatactgcacagaagtagatggagtcttaatgctaggtaagggtaaacaagctgaaatagcagtcagtgacttcagagaccatgaaaccaaagttaatcttctaagtccttttaattgttcttataaactagcataagatataaacttaagtagtacacatgagttttataatttactaatctctgacagatagctaagcatagcacatcagagcataacacagtgtgagggaaataaagtgtacaatgacatcttctattctggacctaataattcaatagagaaagaactacttgtagtcactgtggttacagaaggtttcatggacagcgaacataaagctctactagctaacaaataggtcttaatgataaaaacgtgggccttcagagaactaaaggtaccaatgtgtggcagtccaaaattacgaggaaaatgagttcccttcatgggtcacatcagcaattttttttttccccttttgagacagagtcttgctctgctgcccaggttggagtgcagtggcatgatctaggctcactgcaacctccgcctcccgggttcaagcaattctcatgcctcagcctcccgagtagctgggattacaggtgcctgtcatcacggctggctactttttgtatttttagtagagacagggtttcaccatgttggccaggctggtctcaaactcctgacctcaagtgatctgcttgcttcagcctcccgaagtgctgtgatcgtaggtgtgagccactgtgcccagctacctcatcaattcttaatctataaaccatggataggcttcgggagaacccaagaaccaatgaaatctgttggtaagttttatgtgtgcggttttctacagagagggtcaacagcatgtatattttcaaagaagtctgtggtgcaaaagagagtttattgttagaagtccttgggcaatcaacttggaaaagggtggattgagaatgggggctgtctagatcaggataatgttgaatttgaccctcacttgaggcttttgtacagaggatgagaagacggtaaattcaagggttaatcagaaattaacaccaacatgacttggtgatgagtgagatgtgaaacgtgagaaaaacatcaatgatgaaatcaagcttctgacttgcaacagtgagtataccaagagctacaggcttggaagatgaataaagttgggagcattctgttttttcatgagtgcccatgggacagacagggagaaatggacagttgaaagtacaagtctagacaggcacagtggctcatgtctgtaaccctagcactttgggaggctgagataggagaattactagggttcaggagtttgagacgaacctgggtgacatagtgagagctcatctctacaaaaaataaaattagctcggcatggtgctgcaagattatagtccctgttagtcgagaggctgaggtgggagaactgcttgagcccaggagggaaagcagcagtgaactgagatcacgccactgcactccagcctgggcgacagtgagaccctgtctcaaaaaaaaaaaaaaaaatgcaagtctggagaaatatagctgggagtcagtaatgccagttttagctgagggagttaagatcatttaatcagtgttaaggaagaaactcaatagtagtgaccaccaatacttaaggaaaaaggataaagtaagaggaatgataaaggctggctgaaatatcttggtgtctagcctaagaaaggaggggttagatgctcatgtttattaatatggatctagagaagcatttattcactaatacattttatttgtgttctctaatttaaaattaccttttcatcttgcttgattttccttcagctaaattagaaatttgtagtttttcccctaaaaaattcaatggcattctttcttataaattacattctctgattttcttgtcagcctgcttcaaggaaatccatgtgttcaaaatgcttgctcgcagtttgctccataccaaatggttgcttaacccaaatatctgagcagcaaattgagctgatccttctggagaaagtacggttgaacagccaagaccactgggtagtcgaagagaagaccacacatcctgaactccccagtctggtgtgaggggaggacagctgataactggatatgcagtgttcccagacatcactggtcccaaaccattacttctgcctgccactgccacaaatacagtaggaatgccatccccttcatactcagctttaatcctcagagtttcatctggtcctttatgcgcagatgttactcgaagttcacatggaatgccaaaatttccacaggccttcttgattttttcacagtgaccaagatcagaagtagagcccatcaacactacaaccctgcactgactttctgatttcaaaagcaactctactctctctgcaacccactcaaagtttttctttaccatttggagcccttcaggagttacttctttgaggtcccgataagactgtttgtctttctgttggcttcgatctcctgatggccagagtctccaggaatcattgtcaataacatcagcaagaacaatttctttggtggttacatcaacaccaaattcaatcttcatatcaaccagtgtacaattctggggcaaccaggatttctccagtatttcaaatatagcctgtgtagcatgactcatgatatccacttcagtctggcctataagaagtccagcaaagcaaaattttgcagcaatcagctgttcctcagaccactgtgggtcattattggcatcatccttgaaaaacaactccactttaggtgggtaaaacttatatccttccttgacaccaggatttcttttgagaaaagaaccagttgctattcttctgcaaacccattcaattggaatcatttcacactgcggtgcaatgaaagctgtctccccacattttctggtgaaggcagttttaatacctgcttcctgtaataactgaaaaatacaactggtgattttatttgagattgcagcttttccttccaggtggttttttctagctgcatttcctgctgtaatctggtccttggactgcaggaggacttttcctggactgtctaacaattcgtagacttcttttgttttaccctcatataattttttaccaatgttcagtacctcagctgtcgccattatcctaagtgggctgagggctgcgaccgcgccgggaagcgaggcagaactcaagtcttgacggcctgggggaagcatgcagggaagggcatatgaaggctaaatgctctgaaagagaaatgaggttaagtccgttactcccattacgctactgttgggtgctggaaaataacggagatttccacgtgcagcaaatacagctttccaggcagctcttaggggaaggct

SEQ ID NO: 18360 - RNA, 3447 nt, Homo sapiens
  source 1..3447: mol_type = other RNA
tgaagtaccagctactcgagaggctgcagcttgagtccaggagttcaaggctgcagggagccataatcatgccactgcactccagcctgggagacagtgagaacttggctcttaaaaaaaaaaaggaaaaaaaattgataacgacaatttgtaatggtcagtcctatccaccagtctaaatgaaagtttaaaaattttcatatactgcacagaagtagatggagtcttaatgctaggtaagggtaaacaagctgaaatagcagtcagtgacttcagagaccatgaaaccaaagttaatcttctaagtccttttaattgttcttataaactagcataagatataaacttaagtagtacacatgagttttataatttactaatctctgacagatagctaagcatagcacatcagagcataacacagtgtgagggaaataaagtgtacaatgacatcttctattctggacctaataattcaatagagaaagaactacttgtagtcactgtggttacagaaggtttcatggacagcgaacataaagctctactagctaacaaataggtcttaatgataaaaacgtgggccttcagagaactaaaggtaccaatgtgtggcagtccaaaattacgaggaaaatgagttcccttcatgggtcacatcagcaattttttttttccccttttgagacagagtcttgctctgctgcccaggttggagtgcagtggcatgatctaggctcactgcaacctccgcctcccgggttcaagcaattctcatgcctcagcctcccgagtagctgggattacaggtgcctgtcatcacggctggctactttttgtatttttagtagagacagggtttcaccatgttggccaggctggtctcaaactcctgacctcaagtgatctgcttgcttcagcctcccgaagtgctgtgatcgtaggtgtgagccactgtgcccagctacctcatcaattcttaatctataaaccatggataggcttcgggagaacccaagaaccaatgaaatctgttggtaagttttatgtgtgcggttttctacagagagggtcaacagcatgtatattttcaaagaagtctgtggtgcaaaagagagtttattgttagaagtccttgggcaatcaacttggaaaagggtggattgagaatgggggctgtctagatcaggataatgttgaatttgaccctcacttgaggcttttgtacagaggatgagaagacggtaaattcaagggttaatcagaaattaacaccaacatgacttggtgatgagtgagatgtgaaacgtgagaaaaacatcaatgatgaaatcaagcttctgacttgcaacagtgagtataccaagagctacaggcttggaagatgaataaagttgggagcattctgttttttcatgagtgcccatgggacagacagggagaaatggacagttgaaagtacaagtctagacaggcacagtggctcatgtctgtaaccctagcactttgggaggctgagataggagaattactagggttcaggagtttgagacgaacctgggtgacatagtgagagctcatctctacaaaaaataaaattagctcggcatggtgctgcaagattatagtccctgttagtcgagaggctgaggtgggagaactgcttgagcccaggagggaaagcagcagtgaactgagatcacgccactgcactccagcctgggcgacagtgagaccctgtctcaaaaaaaaaaaaaaaaatgcaagtctggagaaatatagctgggagtcagtaatgccagttttagctgagggagttaagatcatttaatcagtgttaaggaagaaactcaatagtagtgaccaccaatacttaaggaaaaaggataaagtaagaggaatgataaaggctggctgaaatatcttggtgtctagcctaagaaaggaggggttagatgctcatgtttattaatatggatctagagaagcatttattcactaatacattttatttgtgttctctaatttaaaattaccttttcatcttgcttgattttccttcagctaaattagaaatttgtagtttttcccctaaaaaattcaatggcattctttcttataaattacattctctgattttcttgtcagcctgcttcaaggaaatccatgtgttcaaaatgcttgctcgcagtttgctccataccaaatggttgcttaacccaaatatctgagcagcaaattgagctgatccttctggagaaagtacggttgaacagccaagaccactgggtagtcgaagagaagaccacacatcctgaactccccagtctggtgtgaggggaggacagctgataactggatatgcagtgttcccagacatcactggtcccaaaccattacttctgcctgccactgccacaaatacagtaggaatgccatccccttcatactcagctttaatcctcagagtttcatctggtcctttatgcgcagatgttactcgaagttcacatggaatgccaaaatttccacaggccttcttgattttttcacagtgaccaagatcagaagtagagcccatcaacactacaaccctgcactgactttctgatttcaaaagcaactctactctctctgcaacccactcaaagtttttctttaccatttggagcccttcaggagttacttctttgaggtcccgataagactgtttgtctttctgttggcttcgatctcctgatggccagagtctccaggaatcattgtcaataacatcagcaagaacaatttctttggtggttacatcaacaccaaattcaatcttcatatcaaccagtgtacaattctggggcaaccaggatttctccagtatttcaaatatagcctgtgtagcatgactcatgatatccacttcagtctggcctataagaagtccagcaaagcaaaattttgcagcaatcagctgttcctcagaccactgtgggtcattattggcatcatccttgaaaaacaactccactttaggtgggtaaaacttatatccttccttgacaccaggatttcttttgagaaaagaaccagttgctattcttctgcaaacccattcaattggaatcatttcacactgcggtgcaatgaaagctgtctccccacattttctggtgaaggcagttttaatacctgcttcctgtaataactgaaaaatacaactggtgattttatttgagattgcagcttttccttccaggtggttttttctagctgcatttcctgctgtaatctggtccttggactgcaggaggacttttcctggactgtctaacaattcgtagacttcttttgttttaccctcatataattttttaccaatgttcagtacctcagctgtcgccattatcctaagtgggctgagggctgcgaccgcgccgggaagcgaggcagaactct

SEQ ID NO: 18361 - RNA, 3468 nt, Homo sapiens
  source 1..3468: mol_type = other RNA
tgaagtaccagctactcgagaggctgcagcttgagtccaggagttcaaggctgcagggagccataatcatgccactgcactccagcctgggagacagtgagaacttggctcttaaaaaaaaaaaggaaaaaaaattgataacgacaatttgtaatggtcagtcctatccaccagtctaaatgaaagtttaaaaattttcatatactgcacagaagtagatggagtcttaatgctaggtaagggtaaacaagctgaaatagcagtcagtgacttcagagaccatgaaaccaaagttaatcttctaagtccttttaattgttcttataaactagcataagatataaacttaagtagtacacatgagttttataatttactaatctctgacagatagctaagcatagcacatcagagcataacacagtgtgagggaaataaagtgtacaatgacatcttctattctggacctaataattcaatagagaaagaactacttgtagtcactgtggttacagaaggtttcatggacagcgaacataaagctctactagctaacaaataggtcttaatgataaaaacgtgggccttcagagaactaaaggtaccaatgtgtggcagtccaaaattacgaggaaaatgagttcccttcatgggtcacatcagcaattttttttttccccttttgagacagagtcttgctctgctgcccaggttggagtgcagtggcatgatctaggctcactgcaacctccgcctcccgggttcaagcaattctcatgcctcagcctcccgagtagctgggattacaggtgcctgtcatcacggctggctactttttgtatttttagtagagacagggtttcaccatgttggccaggctggtctcaaactcctgacctcaagtgatctgcttgcttcagcctcccgaagtgctgtgatcgtaggtgtgagccactgtgcccagctacctcatcaattcttaatctataaaccatggataggcttcgggagaacccaagaaccaatgaaatctgttggtaagttttatgtgtgcggttttctacagagagggtcaacagcatgtatattttcaaagaagtctgtggtgcaaaagagagtttattgttagaagtccttgggcaatcaacttggaaaagggtggattgagaatgggggctgtctagatcaggataatgttgaatttgaccctcacttgaggcttttgtacagaggatgagaagacggtaaattcaagggttaatcagaaattaacaccaacatgacttggtgatgagtgagatgtgaaacgtgagaaaaacatcaatgatgaaatcaagcttctgacttgcaacagtgagtataccaagagctacaggcttggaagatgaataaagttgggagcattctgttttttcatgagtgcccatgggacagacagggagaaatggacagttgaaagtacaagtctagacaggcacagtggctcatgtctgtaaccctagcactttgggaggctgagataggagaattactagggttcaggagtttgagacgaacctgggtgacatagtgagagctcatctctacaaaaaataaaattagctcggcatggtgctgcaagattatagtccctgttagtcgagaggctgaggtgggagaactgcttgagcccaggagggaaagcagcagtgaactgagatcacgccactgcactccagcctgggcgacagtgagaccctgtctcaaaaaaaaaaaaaaaaatgcaagtctggagaaatatagctgggagtcagtaatgccagttttagctgagggagttaagatcatttaatcagtgttaaggaagaaactcaatagtagtgaccaccaatacttaaggaaaaaggataaagtaagaggaatgataaaggctggctgaaatatcttggtgtctagcctaagaaaggaggggttagatgctcatgtttattaatatggatctagagaagcatttattcactaatacattttatttgtgttctctaatttaaaattaccttttcatcttgcttgattttccttcagctaaattagaaatttgtagtttttcccctaaaaaattcaatggcattctttcttataaattacattctctgattttcttgtcagcctgcttcaaggaaatccatgtgttcaaaatgcttgctcgcagtttgctccataccaaatggttgcttaacccaaatatctgagcagcaaattgagctgatccttctggagaaagtacggttgaacagccaagaccactgggtagtcgaagagaagaccacacatcctgaactccccagtctggtgtgaggggaggacagctgataactggatatgcagtgttcccagacatcactggtcccaaaccattacttctgcctgccactgccacaaatacagtaggaatgccatccccttcatactcagctttaatcctcagagtttcatctggtcctttatgcgcagatgttactcgaagttcacatggaatgccaaaatttccacaggccttcttgattttttcacagtgaccaagatcagaagtagagcccatcaacactacaaccctgcactgactttctgatttcaaaagcaactctactctctctgcaacccactcaaagtttttctttaccatttggagcccttcaggagttacttctttgaggtcccgataagactgtttgtctttctgttggcttcgatctcctgatggccagagtctccaggaatcattgtcaataacatcagcaagaacaatttctttggtggttacatcaacaccaaattcaatcttcatatcaaccagtgtacaattctggggcaaccaggatttctccagtatttcaaatatagcctgtgtagcatgactcatgatatccacttcagtctggcctataagaagtccagcaaagcaaaattttgcagcaatcagctgttcctcagaccactgtgggtcattattggcatcatccttgaaaaacaactccactttaggtgggtaaaacttatatccttccttgacaccaggatttcttttgagaaaagaaccagttgctattcttctgcaaacccattcaattggaatcatttcacactgcggtgcaatgaaagctgtctccccacattttctggtgaaggcagttttaatacgatttgacttatatgaggtaactgcttcctgtaataactgaaaaatacaactggtgattttatttgagattgcagcttttccttccaggtggttttttctagctgcatttcctgctgtaatctggtccttggactgcaggaggacttttcctggactgtctaacaattcgtagacttcttttgttttaccctcatataattttttaccaatgttcagtacctcagctgtcgccattatcctaagtgggctgagggctgcgaccgcgccgggaagcgaggcagaactct

SEQ ID NO: 18362 - RNA, 215 nt, Homo sapiens
  source 1..215: mol_type = other RNA
tgaagtaccagctactcgagaggctggggtgggagaatcacttgaaccagggaggtggaggttgcagtgaactgggatcgtgccagcctgggcgacagagtgagacccgcagctctggcctccgttcccctcgcgccccctcagcagtgcctcttcctacactccgccgccgccgccgccgccatcttccgttcgtcgccgggaacggtgcgcac

SEQ ID NO: 18363 - RNA, 6438 nt, Homo sapiens
  source 1..6438: mol_type = other RNA
tgaagtaccagctactcgagaggcttaggcaggagaattgcttgaacccgggaggtggaggttgcggtgagctaagttcaggccactgcactccagcctgggcaagacagtgagactctgtctcaaaaaataataataataaataaacataaaaataaaaactgatatggtaatgcctaaaatatttttaggggataaggccacaaaataacctggattttcatattaagccaccaactcttcatgtagaagagagtaaaggtggttaaaaaaaagggggggaatgcctaaacacatgggcaaaattattttcccctttaagatctaataaggctaacccaaaaaacctagagactgtatgtgtgcatgtgtccaaatgataaaagttagagacttgcagatccaatttaaatgaagcaggaggagtttgtgctatgcataaaaaaaatcaccagtttttaaaaactgtattaaagattatggaatctcattttctggaatgctttaaaaagaaagaaaacttatattttgtttgtattcatttaagtcaaccccattcaaaagttgacataattcattataattccttctttttaataagtttgctatattcattctcacaatgttaaatttgctggcatgagagagataatcataaaaaataagagggatatgatttgaggaacaaaattctatatacggtgctaaattattttgtgacataaattaagatgaagttcttctacagaaaatgttggacaaaggctgtttctgaatcttaaaatgaaaggactctaaacactaattttaaatgaatataaaaattctgaaaaataatatttatagcaaaatagttcaagattagttttctcaccaaagctgggaaagctgtgtgcacaaagtaccaaatatatttcaactgaagtactgaatcctcaactagcctgaacacaaaaccaacttctattttacctcattacctctcagtttgtttgctagccgagtcatcattctctcacgttgttgtaaacaagatgagcttctcagatcatatgctctcacaggtgtagaaggacctttctgtcggccatggtagctttcatcagtcttcttcctccttcttgcaacgcggcaagaagcccgcacaggtcgctttggaggaggatttgccatagcgcttgacagctcttcggcaccagctggtggaactgaagagttcaaaagcactttagctgttctcttcgccttctttagcctactgacaacagattttttcttcttcagataccttccaagaaaagcgctcctggactgatatctatgacgtaaaaagacagagtatttcgaaatatactttctaatgatatcacttggtttggtccgaatccaaattgactgtttctctgaagcttttctgggtttttgctggagaataattggtttataaacctttttgggaaaacctagcttattactactagttgtcaccctctttccatgaattttctttttactttgactttccaaaagcttatttctaactgattttggagagattttgacaacatcatgatttaaaaatgttagctggaaatttcttttctttggaagctcacgagcatgcagaacctttgattcttccagaaacagagaagagtcactggttccctgatgtgaattaaatccatatcttgccggcactgccattaaaggcgctgaagcagagccttgtccatcagcatcattatctcctgcactggagttttggttgctcctattaaaatgaattttaacccagttacgcctctcaaactctggtactattacactcaggggaggactaattacaatttgcttaatcaagggctcataataatcaaagatattccgtttatatttgcatataaaccgaatatcattatcccaactatggtgcctcattttagggaaaggaaggccttcaccctctttcagtttaatatttaaagaagaaagaacacagactaaggctttgggttgcataggcttcaaaactttagtacatgatgcaggaaattcaactgtcccaattttgactttctttttggtttttctgtcatcctgtaaacgtgaacacttactttttggtgggtcttcctcttgtctaattatttttcttttcatcactgggtaattcttacaactggtctgagtactatggctgattttcgctgtctggcattgagaagccacacgccccttttgcttaggaggcctctctgctggaggatgacgatggcatggtttatctaaggccactgacaagtcatcaatatctgaaataccacagacaatatcatcactctctgacacagcttgagttggtgcagtgtcctccttaccttgcaagtcagcccaggtaaccttttttttccccttcgaagaaacttttttggtctcacagtcatcatcaaagtaacagtggaaacgaccttccctaaactccttcaccagagcattaatttttatgtcatcttctctcattatctgagaccatgttttccccacaaatgaaggaggtacatgaggcaaggcttcaagaactggttcatcaggattatcctctatgacatcctttgcttttttcaggttccttacagaatcaaccttgagaacagagcttgactgggaatcatggttcttttctttcaagtcagaagataccttcttacaagggtgtcttttcttaacagtttcttgaggctgatcagtatcagatggaagagggggagcacactgaaaattcatctcaaaaccatccggttcacagctcacttctagatctctatgttttagcttcgaacgtttttttttatcagcccttcgatggagcgctgacttggaagaggcaccaaaatccactgcagaagcactagactgacagctcttaccttttaggccagcatttcttggatccttccgaagactggcttctttgtgagctttctgcagtcggtgagtcgttcgatgagaagtgtcttccaaattaaattttcctttagaaccattatatccacagctcttatcttctgaatcaatatatttcaccattttctcatcaggtccttgtgactcgtaagtcatggactgatcagaggcatcaacattaaaattcatttcagaaccacaagattgacaacttggctctcccagaataatatagtccttcttccggtttattattttgaaagtctctttgcattggtttgtcattgagggagtagaggctttacaattacatctgacttcagaaccaaaaaagtcacagctcttatcttctatatcaatacattctgtatttatacagctgatatctttgacagtcaactgaggtgggtcagtcactaactgaaggggaatatcatctgaaattacttcataatcactatcaccgggcaccagatccacaagtaccacctttggaaggtgggtttctttgactgatcctggaaattggttaactactatttgaaaaggaacatcagaatcatacatcatttctgaatcactaggttgatcggtcttttcttccatgacaacatgctcttccttctgaaggtctgcctctttgtaagacacttgaggttggtcaacttctgactgaagatgaacacaagaatgacattttatttcagaaccacagacttcacagttcttattttctagatcattatgatccttcttttgcaagtttatttctttgacaggtacagaagattgatcagtcacaaactgaacaggaatatgagaagcataacttacatcaaaatcacctaatttatagctcttatcttccaggtaaatatggtcttccttccaaagatttatttctttgacaggtttttgaagctcatctgctgctgcctgaaaagagtcattggaatcagaactttcttcaggactataagaattactgctcttatcttccagactggcatgctcctcttccaaaatgtgtggttgttttatcactgactgaagagggatatttgaaacataaattatttcagaatcactgggcacatagcccttatcatccagacaaacatgttcctccctcaaaagatttatttctttattcgcccctggaattttattagttacggactgaaggggttcatgagaatcaaaatttattctggaatctgtaggtttgacaatcttattttccaagtcaacatgctctttccaaagactgacctccttaactacttcttcaggttggccagccactggctgaagaacatcagaatcatacataatttcaaaacccttagcttcatttctcctatcttccgtgtcaacttcttcatccttccaaaggcttatttctttaacggtttctctcagccggtcagccactgactgaagagggtcatcagaatcaaaacttacttcagaaccacaacattgattgtgcttaccttctagttcaatgtgctcctgctccaaaatagttatttgaggtcgattgactattgactgacccaagaaaccagaatccaaattcatttctgaacaactatattggctgttcttaacttccaagtacatatggttttcattcccaaggttcacatgtttaatagctactttgggttgatcagccacagattggacagaaacatcaggatgatgtattaatttataagtactaggttcattaatcttatttttcaggccaataacctcttccttccattggtctatttttttaaccgcttcctgaagttgttcagaatcaaaagttattttagaatcacctgatttactgtttttgtccttcagattaacatgtttttccttcaaaaaagctagttgaggttggtcagtcattgactgaggtggaacattagaatccaaaattatttcagaaccactacatttatcattcttgttttctagaacatattgcttctttctgtttattttgttaacagctacttgaggttcagttactgaataatgagggacaccagaatctaaacttgtttttgaaccactgaattcagtacttctaccttggaattcagcgtgcttttctctttgaagccatgtttctttgacaattacttcaggtttgtgagtcgctgcctgaagagggacatcagaatccaaacttgtttcaaaaacactcttattttctaagtacatgtgctcttttgtgtgaaggcttatttctttaatgggatcttcagaacgtccagtcactgaatgaaaaatgatattataatccaaacttacttcagaatcaataggttcattttccttattttctaagtgtacctgctcttctttttgaggatttagctttttaacagctacttcgggagaattagtcactgaatgaagaggggcatgggaatccgaacttatttcagaaccactgggttcatcattcttcctttctaagtgaatgtactcttctttctgaattacttctttaacagctacttcagggtgatcatttcagctctcatcttccaggtcaatgtgccgttcttttccttcagcatccagatgagactgctcagtaactgacagaagaggcgggtcagaatcaaaagtcaactcagagctggagcaatcatagctcctaacttccatgtcaatatttaactctttaagatttacttcatccaaagcttcttgaggctcatcatgagctgaatgataaagagaagccggagaatcagaactcagagaagaacggctagactgaacactcttattctcaaggtcaacatccactttctgacgctctatttcggctacttgagactggtcagctaattgagcatcagcctgaaaacccatttcaggaccatgggattcacagttcatatccataaggtcagcattcttctccttcagaagatttatcttttcaacagccctctgggattcatctgcaactgtcccaagtgagacatcacaatcaagatgtgctttagcactactgggtttacgcttcttatgttttaggtggacttgtctacctttcaggtttcttcctttgacagtcagttggggatgatcaactactgactcaagagaaacatcacaatcaaaacttgtttcagaacaactcgatccatagttatcaaccaagctggtatgagccttcttccgaagttttgtttctgtgacagccactgggggtctgtcaaccactgactgcagtgggaaaacagaatcagcacttacttcagagctactggaaccatagttcttatcaaccaaaccaatgtgcacttccttaggaaggtttacttctgttacagattgttgggggtagtcactagtggactgaggtgaagcatcacaatcaaaattcgtttcagaactactagattcatagctttggtcaaccaggctaatatgccttgcattctgaag

SEQ ID NO: 18364 - RNA, 9580 nt, Homo sapiens
  source 1..9580: mol_type = other RNA
tgaagtaccagctactcgagaggcttaggcaggagaattgcttgaacccgggaggtggaggttgcggtgagctaagttcaggccactgcactccagcctgggcaagacagtgagactctgtctcaaaaaataataataataaataaacataaaaataaaaactgatatggtaatgcctaaaatatttttaggggataaggccacaaaataacctggattttcatattaagccaccaactcttcatgtagaagagagtaaaggtggttaaaaaaaagggggggaatgcctaaacacatgggcaaaattattttcccctttaagatctaataaggctaacccaaaaaacctagagactgtatgtgtgcatgtgtccaaatgataaaagttagagacttgcagatccaatttaaatgaagcaggaggagtttgtgctatgcataaaaaaaatcaccagtttttaaaaactgtattaaagattatggaatctcattttctggaatgctttaaaaagaaagaaaacttatattttgtttgtattcatttaagtcaaccccattcaaaagttgacataattcattataattccttctttttaataagtttgctatattcattctcacaatgttaaatttgctggcatgagagagataatcataaaaaataagagggatatgatttgaggaacaaaattctatatacggtgctaaattattttgtgacataaattaagatgaagttcttctacagaaaatgttggacaaaggctgtttctgaatcttaaaatgaaaggactctaaacactaattttaaatgaatataaaaattctgaaaaataatatttatagcaaaatagttcaagattagttttctcaccaaagctgggaaagctgtgtgcacaaagtaccaaatatatttcaactgaagtactgaatcctcaactagcctgaacacaaaaccaacttctattttacctcattacctctcagtttgtttgctagccgagtcatcattctctcacgttgttgtaaacaagatgagcttctcagatcatatgctctcacaggtgtagaaggacctttctgtcggccatggtagctttcatcagtcttcttcctccttcttgcaacgcggcaagaagcccgcacaggtcgctttggaggaggatttgccatagcgcttgacagctcttcggcaccagctggtggaactgaagagttcaaaagcactttagctgttctcttcgccttctttagcctactgacaacagattttttcttcttcagataccttccaagaaaagcgctcctggactgatatctatgacgtaaaaagacagagtatttcgaaatatactttctaatgatatcacttggtttggtccgaatccaaattgactgtttctctgaagcttttctgggtttttgctggagaataattggtttataaacctttttgggaaaacctagcttattactactagttgtcaccctctttccatgaattttctttttactttgactttccaaaagcttatttctaactgattttggagagattttgacaacatcatgatttaaaaatgttagctggaaatttcttttctttggaagctcacgagcatgcagaacctttgattcttccagaaacagagaagagtcactggttccctgatgtgaattaaatccatatcttgccggcactgccattaaaggcgctgaagcagagccttgtccatcagcatcattatctcctgcactggagttttggttgctcctattaaaatgaattttaacccagttacgcctctcaaactctggtactattacactcaggggaggactaattacaatttgcttaatcaagggctcataataatcaaagatattccgtttatatttgcatataaaccgaatatcattatcccaactatggtgcctcattttagggaaaggaaggccttcaccctctttcagtttaatatttaaagaagaaagaacacagactaaggctttgggttgcataggcttcaaaactttagtacatgatgcaggaaattcaactgtcccaattttgactttctttttggtttttctgtcatcctgtaaacgtgaacacttactttttggtgggtcttcctcttgtctaattatttttcttttcatcactgggtaattcttacaactggtctgagtactatggctgattttcgctgtctggcattgagaagccacacgccccttttgcttaggaggcctctctgctggaggatgacgatggcatggtttatctaaggccactgacaagtcatcaatatctgaaataccacagacaatatcatcactctctgacacagcttgagttggtgcagtgtcctccttaccttgcaagtcagcccaggtaaccttttttttccccttcgaagaaacttttttggtctcacagtcatcatcaaagtaacagtggaaacgaccttccctaaactccttcaccagagcattaatttttatgtcatcttctctcattatctgagaccatgttttccccacaaatgaaggaggtacatgaggcaaggcttcaagaactggttcatcaggattatcctctatgacatcctttgcttttttcaggttccttacagaatcaaccttgagaacagagcttgactgggaatcatggttcttttctttcaagtcagaagataccttcttacaagggtgtcttttcttaacagtttcttgaggctgatcagtatcagatggaagagggggagcacactgaaaattcatctcaaaaccatccggttcacagctcacttctagatctctatgttttagcttcgaacgtttttttttatcagcccttcgatggagcgctgacttggaagaggcaccaaaatccactgcagaagcactagactgacagctcttaccttttaggccagcatttcttggatccttccgaagactggcttctttgtgagctttctgcagtcggtgagtcgttcgatgagaagtgtcttccaaattaaattttcctttagaaccattatatccacagctcttatcttctgaatcaatatatttcaccattttctcatcaggtccttgtgactcgtaagtcatggactgatcagaggcatcaacattaaaattcatttcagaaccacaagattgacaacttggctctcccagaataatatagtccttcttccggtttattattttgaaagtctctttgcattggtttgtcattgagggagtagaggctttacaattacatctgacttcagaaccaaaaaagtcacagctcttatcttctatatcaatacattctgtatttatacagctgatatctttgacagtcaactgaggtgggtcagtcactaactgaaggggaatatcatctgaaattacttcataatcactatcaccgggcaccagatccacaagtaccacctttggaaggtgggtttctttgactgatcctggaaattggttaactactatttgaaaaggaacatcagaatcatacatcatttctgaatcactaggttgatcggtcttttcttccatgacaacatgctcttccttctgaaggtctgcctctttgtaagacacttgaggttggtcaacttctgactgaagatgaacacaagaatgacattttatttcagaaccacagacttcacagttcttattttctagatcattatgatccttcttttgcaagtttatttctttgacaggtacagaagattgatcagtcacaaactgaacaggaatatgagaagcataacttacatcaaaatcacctaatttatagctcttatcttccaggtaaatatggtcttccttccaaagatttatttctttgacaggtttttgaagctcatctgctgctgcctgaaaagagtcattggaatcagaactttcttcaggactataagaattactgctcttatcttccagactggcatgctcctcttccaaaatgtgtggttgttttatcactgactgaagagggatatttgaaacataaattatttcagaatcactgggcacatagcccttatcatccagacaaacatgttcctccctcaaaagatttatttctttattcgcccctggaattttattagttacggactgaaggggttcatgagaatcaaaatttattctggaatctgtaggtttgacaatcttattttccaagtcaacatgctctttccaaagactgacctccttaactacttcttcaggttggccagccactggctgaagaacatcagaatcatacataatttcaaaacccttagcttcatttctcctatcttccgtgtcaacttcttcatccttccaaaggcttatttctttaacggtttctctcagccggtcagccactgactgaagagggtcatcagaatcaaaacttacttcagaaccacaacattgattgtgcttaccttctagttcaatgtgctcctgctccaaaatagttatttgaggtcgattgactattgactgacccaagaaaccagaatccaaattcatttctgaacaactatattggctgttcttaacttccaagtacatatggttttcattcccaaggttcacatgtttaatagctactttgggttgatcagccacagattggacagaaacatcaggatgatgtattaatttataagtactaggttcattaatcttatttttcaggccaataacctcttccttccattggtctatttttttaaccgcttcctgaagttgttcagaatcaaaagttattttagaatcacctgatttactgtttttgtccttcagattaacatgtttttccttcaaaaaagctagttgaggttggtcagtcattgactgaggtggaacattagaatccaaaattatttcagaaccactacatttatcattcttgttttctagaacatattgcttctttctgtttattttgttaacagctacttgaggttcagttactgaataatgagggacaccagaatctaaacttgtttttgaaccactgaattcagtacttctaccttggaattcagcgtgcttttctctttgaagccatgtttctttgacaattacttcaggtttgtgagtcgctgcctgaagagggacatcagaatccaaacttgtttcaaaaacactcttattttctaagtacatgtgctcttttgtgtgaaggcttatttctttaatgggatcttcagaacgtccagtcactgaatgaaaaatgatattataatccaaacttacttcagaatcaataggttcattttccttattttctaagtgtacctgctcttctttttgaggatttagctttttaacagctacttcgggagaattagtcactgaatgaagaggggcatgggaatccgaacttatttcagaaccactgggttcatcattcttcctttctaagtgaatgtactcttctttctgaattacttctttaacagctacttcagggtgatcatttcctgaatgaagaggaatatcagaatcaaaagttatttcagagacacaagattcattacttttactttccagatcaacagtttcttcctcataaacagctacttcaggttggtcaattactgaataaagaggaatatcagaatcaaaagttatttcagaactatctgactcacagctctcatcttccaggtcaatgtgccgttcttttccttcagcatccagatgagactgctcagtaactgacagaagaggcgggtcagaatcaaaagtcaactcagagctggagcaatcatagctcctaacttccatgtcaatatttaactctttaagatttacttcatccaaagcttcttgaggctcatcatgagctgaatgataaagagaagccggagaatcagaactcagagaagaacggctagactgaacactcttattctcaaggtcaacatccactttctgacgctctatttcggctacttgagactggtcagctaattgagcatcagcctgaaaacccatttcaggaccatgggattcacagttcatatccataaggtcagcattcttctccttcagaagatttatcttttcaacagccctctgggattcatctgcaactgtcccaagtgagacatcacaatcaagatgtgctttagcactactgggtttacgcttcttatgttttaggtggacttgtctacctttcaggtttcttcctttgacagtcagttggggatgatcaactactgactcaagagaaacatcacaatcaaaacttgtttcagaacaactcgatccatagttatcaaccaagctggtatgagccttcttccgaagttttgtttctgtgacagccactgggggtctgtcaaccactgactgcagtgggaaaacagaatcagcacttacttcagagctactggaaccatagttcttatcaaccaaaccaatgtgcacttccttaggaaggtttacttctgttacagattgttgggggtagtcactagtggactgaggtgaagcatcacaatcaaaattcgtttcagaactactagattcatagctttggtcaaccaggctaatatgccttgcattctgaagacttatttctttaacaatcatttgggattggttggtaaccaagtgaagaatgtcatcacaatcagaacttattttagaaacataagatttattattcttatactgtacatcagtacgtacttccttggaaaggtttacttctttggcactcactttagattggtcagtcagtgaatgaaaagaggaactgcaatcaaaactcatttctgaacctctagactcatagttatcttcttggtcaatttgctcctccttccaaagacttaagtcttgtgcagtctcttggggctgatcagatgctgactgaagagagatacaatcaaacttcatttcagaactcactgagcacttctgttcccaaaaggctgtcttgttaaaaaccaaatgcttttcttcttgggtacaatccatgttagaaaagaattcctcatggttctttgcaatagtatcttcaaagattcctttattagaaggcatgtcagttttattcgggtttactgctaatttggaaggagatttaactcttaaggagcccttagtacccatgcgttcatggaatttcaagccagctgataaagttttaccctgagattttacatctttccacaaaaccaacttatctgaattcatgcgtaaagatttcctatttgattctttatgtttctgatacgaaaatgaagtagtttctacatgggatgatggcacaggatttctagaggccccatctggctgttcaagatatttctcaactttgtttgggtcacatttgctaactgaatccaaatgagctgctggtggtaaactagttgtattagctgtaactggtctatcgttagagctttcaggtaaacaactagcaggagcattacaaatcactggggggcgtaccaagttgcttctattatttgtagcctgaccaatatctactaggttacattttctcacactggccccaattttatgaacaaactccaagggctgctgctgtcccttctccagtttttgaataactgatggtcgaactgaaacctcctgcgtgccttcctgagatttatgaggtctggaatgtaactcttcaataggttctgaaacctcggatggtctctcttcggtagcatcctcatcctcaaccttatcctcatcctcttcctcttcttcagaaaaagcatcatccaaatgcaccacttcagacgatgacccagtattcacatgtgtctcatcttgtgttgaactgctctcttgacaatgatatgggtggtgctgcagtacatcctgtaagaaacgttccatcaaactactggtacatatttgacgtctactctgtctggtcaaactcctgtgctgagcactgaacaaatgctgttccaggttattatactgcacacggcaataactgcaatatccttgtcttttctgcatcttgaataaataactgaagtcagatggctactgtctttgaatactcaagctattacttcttattatgagaaattgattttctgacttctcacatttatgaggaaaattaatcaattaaaccagcctctggagcagaaaaggtcaggtatttcatcagctgtattagttctggcaagtatctccgcggaggctgcccggattccttccgggccgcggtggagaccgaggaccgagccgggcgctctcccttcttattccggttccgcggcggcgcccgaatcccagaccgtccgagcgccacggccccgctgcccgcggagccagaaataggcgacttcggcccctgcggtccggaggcgagaagcggcgcgggagcgcgtctctcaggacgcgggccccgagtcgcgactccactcacgcaggcatccaaggcaacgtggcgttgcaaccctgatggaggtttgacgtcagggaaggtgcgaaaaccagaccccttctgacgcaggagcggcgggaccgccccctgcccgcccacccactcactcactctcccacccgggcggaggagccccttcctcccctccagaagctcttaaagcggacacttcctccctggtcagggccccactccggagcttgggaaatctatcgcgttccaacaaaaatgactagactcataagcacagttgggacgcgaagtagagaccaaggttttagcgtttgagggtccaaataaaaactgcttgccaattcaaagcaacgtatgaatgtagaaaagaaaacggggctaagagagctagtcgtttccgtttccatgcctatttcatagtgaggtgcatctcacaaaagctgctgttcaatgagcgcttgctctgtgctaggcaccgtttaaggtttctatacattattgcatttcatttcagagtaactctgaatgaatcctattattgtccccctttgacaaattgagaaaactgaggcttaaggaagttaggtattcaaagatctatcctgcacattaaagggttacaaatattaacaaacaacattaggtcatgcaattatattcactgcgctaccccattacgaatatagttgtgagcaaaaacagtttaagtgtaacggagatcacaaacctaaatgaatcacactactgaatatgaaattataatctgcgataagaaggttctgaaacacctaaaccaattttactaaaatggagagaggccctgttgcaaagcttatgtctaatgtaaaaataatcttaaaatgagctactttgctctttggctgtagctgtaattgtcgttaccctttttagtaagcttgtgattttgtccctttaaagaacaacaacaaaaaaacttgcctattgcttttgcgtccattgtttttattctttctgtatttctcagctccttcttcccccactacatctttctctcactttaaagttgggctcctgcaactgttcgatttataacctcccttagatttaacataccaaaaagtacggatttcttttaaggcaagttttttccacatcccaact

SEQ ID NO: 18365 - RNA, 8286 nt, Homo sapiens
  source 1..8286: mol_type = other RNA
tgaagtaccagctactcgagaggcttaggcaggagaattgcttgaacccgggaggtggaggttgcggtgagctaagttcaggccactgcactccagcctgggcaagacagtgagactctgtctcaaaaaataataataataaataaacataaaaataaaaactgatatggtaatgcctaaaatatttttaggggataaggccacaaaataacctggattttcatattaagccaccaactcttcatgtagaagagagtaaaggtggttaaaaaaaagggggggaatgcctaaacacatgggcaaaattattttcccctttaagatctaataaggctaacccaaaaaacctagagactgtatgtgtgcatgtgtccaaatgataaaagttagagacttgcagatccaatttaaatgaagcaggaggagtttgtgctatgcataaaaaaaatcaccagtttttaaaaactgtattaaagattatggaatctcattttctggaatgctttaaaaagaaagaaaacttatattttgtttgtattcatttaagtcaaccccattcaaaagttgacataattcattataattccttctttttaataagtttgctatattcattctcacaatgttaaatttgctggcatgagagagataatcataaaaaataagagggatatgatttgaggaacaaaattctatatacggtgctaaattattttgtgacataaattaagatgaagttcttctacagaaaatgttggacaaaggctgtttctgaatcttaaaatgaaaggactctaaacactaattttaaatgaatataaaaattctgaaaaataatatttatagcaaaatagttcaagattagttttctcaccaaagctgggaaagctgtgtgcacaaagtaccaaatatatttcaactgaagtactgaatcctcaactagcctgaacacaaaaccaacttctattttacctcattacctctcagtttgtttgctagccgagtcatcattctctcacgttgttgtaaacaagatgagcttctcagatcatatgctctcacaggtgtagaaggacctttctgtcggccatggtagctttcatcagtcttcttcctccttcttgcaacgcggcaagaagcccgcacaggtcgctttggaggaggatttgccatagcgcttgacagctcttcggcaccagctggtggaactgaagagttcaaaagcactttagctgttctcttcgccttctttagcctactgacaacagattttttcttcttcagataccttccaagaaaagcgctcctggactgatatctatgacgtaaaaagacagagtatttcgaaatatactttctaatgatatcacttggtttggtccgaatccaaattgactgtttctctgaagcttttctgggtttttgctggagaataattggtttataaacctttttgggaaaacctagcttattactactagttgtcaccctctttccatgaattttctttttactttgactttccaaaagcttatttctaactgattttggagagattttgacaacatcatgatttaaaaatgttagctggaaatttcttttctttggaagctcacgagcatgcagaacctttgattcttccagaaacagagaagagtcactggttccctgatgtgaattaaatccatatcttgccggcactgccattaaaggcgctgaagcagagccttgtccatcagcatcattatctcctgcactggagttttggttgctcctattaaaatgaattttaacccagttacgcctctcaaactctggtactattacactcaggggaggactaattacaatttgcttaatcaagggctcataataatcaaagatattccgtttatatttgcatataaaccgaatatcattatcccaactatggtgcctcattttagggaaaggaaggccttcaccctctttcagtttaatatttaaagaagaaagaacacagactaaggctttgggttgcataggcttcaaaactttagtacatgatgcaggaaattcaactgtcccaattttgactttctttttggtttttctgtcatcctgtaaacgtgaacacttactttttggtgggtcttcctcttgtctaattatttttcttttcatcactgggtaattcttacaactggtctgagtactatggctgattttcgctgtctggcattgagaagccacacgccccttttgcttaggaggcctctctgctggaggatgacgatggcatggtttatctaaggccactgacaagtcatcaatatctgaaataccacagacaatatcatcactctctgacacagcttgagttggtgcagtgtcctccttaccttgcaagtcagcccaggtaaccttttttttccccttcgaagaaacttttttggtctcacagtcatcatcaaagtaacagtggaaacgaccttccctaaactccttcaccagagcattaatttttatgtcatcttctctcattatctgagaccatgttttccccacaaatgaaggaggtacatgaggcaaggcttcaagaactggttcatcaggattatcctctatgacatcctttgcttttttcaggttccttacagaatcaaccttgagaacagagcttgactgggaatcatggttcttttctttcaagtcagaagataccttcttacaagggtgtcttttcttaacagtttcttgaggctgatcagtatcagatggaagagggggagcacactgaaaattcatctcaaaaccatccggttcacagctcacttctagatctctatgttttagcttcgaacgtttttttttatcagcccttcgatggagcgctgacttggaagaggcaccaaaatccactgcagaagcactagactgacagctcttaccttttaggccagcatttcttggatccttccgaagactggcttctttgtgagctttctgcagtcggtgagtcgttcgatgagaagtgtcttccaaattaaattttcctttagaaccattatatccacagctcttatcttctgaatcaatatatttcaccattttctcatcaggtccttgtgactcgtaagtcatggactgatcagaggcatcaacattaaaattcatttcagaaccacaagattgacaacttggctctcccagaataatatagtccttcttccggtttattattttgaaagtctctttgcattggtttgtcattgagggagtagaggctttacaattacatctgacttcagaaccaaaaaagtcacagctcttatcttctatatcaatacattctgtatttatacagctgatatctttgacagtcaactgaggtgggtcagtcactaactgaaggggaatatcatctgaaattacttcataatcactatcaccgggcaccagatccacaagtaccacctttggaaggtgggtttctttgactgatcctggaaattggttaactactatttgaaaaggaacatcagaatcatacatcatttctgaatcactaggttgatcggtcttttcttccatgacaacatgctcttccttctgaaggtctgcctctttgtaagacacttgaggttggtcaacttctgactgaagatgaacacaagaatgacattttatttcagaaccacagacttcacagttcttattttctagatcattatgatccttcttttgcaagtttatttctttgacaggtacagaagattgatcagtcacaaactgaacaggaatatgagaagcataacttacatcaaaatcacctaatttatagctcttatcttccaggtaaatatggtcttccttccaaagatttatttctttgacaggtttttgaagctcatctgctgctgcctgaaaagagtcattggaatcagaactttcttcaggactataagaattactgctcttatcttccagactggcatgctcctcttccaaaatgtgtggttgttttatcactgactgaagagggatatttgaaacataaattatttcagaatcactgggcacatagcccttatcatccagacaaacatgttcctccctcaaaagatttatttctttattcgcccctggaattttattagttacggactgaaggggttcatgagaatcaaaatttattctggaatctgtaggtttgacaatcttattttccaagtcaacatgctctttccaaagactgacctccttaactacttcttcaggttggccagccactggctgaagaacatcagaatcatacataatttcaaaacccttagcttcatttctcctatcttccgtgtcaacttcttcatccttccaaaggcttatttctttaacggtttctctcagccggtcagccactgactgaagagggtcatcagaatcaaaacttacttcagaaccacaacattgattgtgcttaccttctagttcaatgtgctcctgctccaaaatagttatttgaggtcgattgactattgactgacccaagaaaccagaatccaaattcatttctgaacaactatattggctgttcttaacttccaagtacatatggttttcattcccaaggttcacatgtttaatagctactttgggttgatcagccacagattggacagaaacatcaggatgatgtattaatttataagtactaggttcattaatcttatttttcaggccaataacctcttccttccattggtctatttttttaaccgcttcctgaagttgttcagaatcaaaagttattttagaatcacctgatttactgtttttgtccttcagattaacatgtttttccttcaaaaaagctagttgaggttggtcagtcattgactgaggtggaacattagaatccaaaattatttcagaaccactacatttatcattcttgttttctagaacatattgcttctttctgtttattttgttaacagctacttgaggttcagttactgaataatgagggacaccagaatctaaacttgtttttgaaccactgaattcagtacttctaccttggaattcagcgtgcttttctctttgaagccatgtttctttgacaattacttcaggtttgtgagtcgctgcctgaagagggacatcagaatccaaacttgtttcaaaaacactcttattttctaagtacatgtgctcttttgtgtgaaggcttatttctttaatgggatcttcagaacgtccagtcactgaatgaaaaatgatattataatccaaacttacttcagaatcaataggttcattttccttattttctaagtgtacctgctcttctttttgaggatttagctttttaacagctacttcgggagaattagtcactgaatgaagaggggcatgggaatccgaacttatttcagaaccactgggttcatcattcttcctttctaagtgaatgtactcttctttctgaattacttctttaacagctacttcagggtgatcatttcctgaatgaagaggaatatcagaatcaaaagttatttcagagacacaagattcattacttttactttccagatcaacagtttcttcctcataaacagctacttcaggttggtcaattactgaataaagaggaatatcagaatcaaaagttatttcagaactatctgactcacagctctcatcttccaggtcaatgtgccgttcttttccttcagcatccagatgagactgctcagtaactgacagaagaggcgggtcagaatcaaaagtcaactcagagctggagcaatcatagctcctaacttccatgtcaatatttaactctttaagatttacttcatccaaagcttcttgaggctcatcatgagctgaatgataaagagaagccggagaatcagaactcagagaagaacggctagactgaacactcttattctcaaggtcaacatccactttctgacgctctatttcggctacttgagactggtcagctaattgagcatcagcctgaaaacccatttcaggaccatgggattcacagttcatatccataaggtcagcattcttctccttcagaagatttatcttttcaacagccctctgggattcatctgcaactgtcccaagtgagacatcacaatcaagatgtgctttagcactactgggtttacgcttcttatgttttaggtggacttgtctacctttcaggtttcttcctttgacagtcagttggggatgatcaactactgactcaagagaaacatcacaatcaaaacttgtttcagaacaactcgatccatagttatcaaccaagctggtatgagccttcttccgaagttttgtttctgtgacagccactgggggtctgtcaaccactgactgcagtgggaaaacagaatcagcacttacttcagagctactggaaccatagttcttatcaaccaaaccaatgtgcacttccttaggaaggtttacttctgttacagattgttgggggtagtcactagtggactgaggtgaagcatcacaatcaaaattcgtttcagaactactagattcatagctttggtcaaccaggctaatatgccttgcattctgaagacttatttctttaacaatcatttgggattggttggtaaccaagtgaagaatgtcatcacaatcagaacttattttagaaacataagatttattattcttatactgtacatcagtacgtacttccttggaaaggtttacttctttggcactcactttagattggtcagtcagtgaatgaaaagaggaactgcaatcaaaactcatttctgaacctctagactcatagttatcttcttggtcaatttgctcctccttccaaagacttaagtcttgtgcagtctcttggggctgatcagatgctgactgaagagagatacaatcaaacttcatttcagaactcactgagcacttctgttcccaaaaggctgtcttgttaaaaaccaaatgcttttcttcttgggtacaatccatgttagaaaagaattcctcatggttctttgcaatagtatcttcaaagattcctttattagaaggcatgtcagttttattcgggtttactgctaatttggaaggagatttaactcttaaggagcccttagtacccatgcgttcatggaatttcaagccagctgataaagttttaccctgagattttacatctttccacaaaaccaacttatctgaattcatgcgtaaagatttcctatttgattctttatgtttctgatacgaaaatgaagtagtttctacatgggatgatggcacaggatttctagaggccccatctggctgttcaagatatttctcaactttgtttgggtcacatttgctaactgaatccaaatgagctgctggtggtaaactagttgtattagctgtaactggtctatcgttagagctttcaggtaaacaactagcaggagcattacaaatcactggggggcgtaccaagttgcttctattatttgtagcctgaccaatatctactaggttacattttctcacactggccccaattttatgaacaaactccaagggctgctgctgtcccttctccagtttttgaataactgatggtcgaactgaaacctcctgcgtgccttcctgagatttatgaggtctggaatgtaactcttcaataggttctgaaacctcggatggtctctcttcggtagcatcctcatcctcaaccttatcctcatcctcttcctcttcttcagaaaaagcatcatccaaatgcaccacttcagacgatgacccagtattcacatgtgtctcatcttgtgttgaactgctctcttgacaatgatatgggtggtgctgcagtacatcctgtaagaaacgttccatcaaactactggtacatatttgacgtctactctgtctggtcaaactcctgtgctgagcactgaacaaatgctgttccaggttattatactgcacacggcaataactgcaatatccttgtcttttctgcatcttgaataaataactgaagtcagatggctactgtctttgaatactcaagctattacttcttattatgagaaattgattttctgacttctcacatttatgaggaaaattaatcaattaaaccagcctctggagcagaaaaggtcaggtatttcatcagctgtattagttctggcaagtatctgcgaggcggccgcgggagcccagcgagcggtcctggcgtccctcgggaagaaggcgccccgggcgcccggcgagcag

SEQ ID NO: 18366 - RNA, 8414 nt, Homo sapiens
  source 1..8414: mol_type = other RNA
tgaagtaccagctactcgagaggcttaggcaggagaattgcttgaacccgggaggtggaggttgcggtgagctaagttcaggccactgcactccagcctgggcaagacagtgagactctgtctcaaaaaataataataataaataaacataaaaataaaaactgatatggtaatgcctaaaatatttttaggggataaggccacaaaataacctggattttcatattaagccaccaactcttcatgtagaagagagtaaaggtggttaaaaaaaagggggggaatgcctaaacacatgggcaaaattattttcccctttaagatctaataaggctaacccaaaaaacctagagactgtatgtgtgcatgtgtccaaatgataaaagttagagacttgcagatccaatttaaatgaagcaggaggagtttgtgctatgcataaaaaaaatcaccagtttttaaaaactgtattaaagattatggaatctcattttctggaatgctttaaaaagaaagaaaacttatattttgtttgtattcatttaagtcaaccccattcaaaagttgacataattcattataattccttctttttaataagtttgctatattcattctcacaatgttaaatttgctggcatgagagagataatcataaaaaataagagggatatgatttgaggaacaaaattctatatacggtgctaaattattttgtgacataaattaagatgaagttcttctacagaaaatgttggacaaaggctgtttctgaatcttaaaatgaaaggactctaaacactaattttaaatgaatataaaaattctgaaaaataatatttatagcaaaatagttcaagattagttttctcaccaaagctgggaaagctgtgtgcacaaagtaccaaatatatttcaactgaagtactgaatcctcaactagcctgaacacaaaaccaacttctattttacctcattacctctcagtttgtttgctagccgagtcatcattctctcacgttgttgtaaacaagatgagcttctcagatcatatgctctcacaggtgtagaaggacctttctgtcggccatggtagctttcatcagtcttcttcctccttcttgcaacgcggcaagaagcccgcacaggtcgctttggaggaggatttgccatagcgcttgacagctcttcggcaccagctggtggaactgaagagttcaaaagcactttagctgttctcttcgccttctttagcctactgacaacagattttttcttcttcagataccttccaagaaaagcgctcctggactgatatctatgacgtaaaaagacagagtatttcgaaatatactttctaatgatatcacttggtttggtccgaatccaaattgactgtttctctgaagcttttctgggtttttgctggagaataattggtttataaacctttttgggaaaacctagcttattactactagttgtcaccctctttccatgaattttctttttactttgactttccaaaagcttatttctaactgattttggagagattttgacaacatcatgatttaaaaatgttagctggaaatttcttttctttggaagctcacgagcatgcagaacctttgattcttccagaaacagagaagagtcactggttccctgatgtgaattaaatccatatcttgccggcactgccattaaaggcgctgaagcagagccttgtccatcagcatcattatctcctgcactggagttttggttgctcctattaaaatgaattttaacccagttacgcctctcaaactctggtactattacactcaggggaggactaattacaatttgcttaatcaagggctcataataatcaaagatattccgtttatatttgcatataaaccgaatatcattatcccaactatggtgcctcattttagggaaaggaaggccttcaccctctttcagtttaatatttaaagaagaaagaacacagactaaggctttgggttgcataggcttcaaaactttagtacatgatgcaggaaattcaactgtcccaattttgactttctttttggtttttctgtcatcctgtaaacgtgaacacttactttttggtgggtcttcctcttgtctaattatttttcttttcatcactgggtaattcttacaactggtctgagtactatggctgattttcgctgtctggcattgagaagccacacgccccttttgcttaggaggcctctctgctggaggatgacgatggcatggtttatctaaggccactgacaagtcatcaatatctgaaataccacagacaatatcatcactctctgacacagcttgagttggtgcagtgtcctccttaccttgcaagtcagcccaggtaaccttttttttccccttcgaagaaacttttttggtctcacagtcatcatcaaagtaacagtggaaacgaccttccctaaactccttcaccagagcattaatttttatgtcatcttctctcattatctgagaccatgttttccccacaaatgaaggaggtacatgaggcaaggcttcaagaactggttcatcaggattatcctctatgacatcctttgcttttttcaggttccttacagaatcaaccttgagaacagagcttgactgggaatcatggttcttttctttcaagtcagaagataccttcttacaagggtgtcttttcttaacagtttcttgaggctgatcagtatcagatggaagagggggagcacactgaaaattcatctcaaaaccatccggttcacagctcacttctagatctctatgttttagcttcgaacgtttttttttatcagcccttcgatggagcgctgacttggaagaggcaccaaaatccactgcagaagcactagactgacagctcttaccttttaggccagcatttcttggatccttccgaagactggcttctttgtgagctttctgcagtcggtgagtcgttcgatgagaagtgtcttccaaattaaattttcctttagaaccattatatccacagctcttatcttctgaatcaatatatttcaccattttctcatcaggtccttgtgactcgtaagtcatggactgatcagaggcatcaacattaaaattcatttcagaaccacaagattgacaacttggctctcccagaataatatagtccttcttccggtttattattttgaaagtctctttgcattggtttgtcattgagggagtagaggctttacaattacatctgacttcagaaccaaaaaagtcacagctcttatcttctatatcaatacattctgtatttatacagctgatatctttgacagtcaactgaggtgggtcagtcactaactgaaggggaatatcatctgaaattacttcataatcactatcaccgggcaccagatccacaagtaccacctttggaaggtgggtttctttgactgatcctggaaattggttaactactatttgaaaaggaacatcagaatcatacatcatttctgaatcactaggttgatcggtcttttcttccatgacaacatgctcttccttctgaaggtctgcctctttgtaagacacttgaggttggtcaacttctgactgaagatgaacacaagaatgacattttatttcagaaccacagacttcacagttcttattttctagatcattatgatccttcttttgcaagtttatttctttgacaggtacagaagattgatcagtcacaaactgaacaggaatatgagaagcataacttacatcaaaatcacctaatttatagctcttatcttccaggtaaatatggtcttccttccaaagatttatttctttgacaggtttttgaagctcatctgctgctgcctgaaaagagtcattggaatcagaactttcttcaggactataagaattactgctcttatcttccagactggcatgctcctcttccaaaatgtgtggttgttttatcactgactgaagagggatatttgaaacataaattatttcagaatcactgggcacatagcccttatcatccagacaaacatgttcctccctcaaaagatttatttctttattcgcccctggaattttattagttacggactgaaggggttcatgagaatcaaaatttattctggaatctgtaggtttgacaatcttattttccaagtcaacatgctctttccaaagactgacctccttaactacttcttcaggttggccagccactggctgaagaacatcagaatcatacataatttcaaaacccttagcttcatttctcctatcttccgtgtcaacttcttcatccttccaaaggcttatttctttaacggtttctctcagccggtcagccactgactgaagagggtcatcagaatcaaaacttacttcagaaccacaacattgattgtgcttaccttctagttcaatgtgctcctgctccaaaatagttatttgaggtcgattgactattgactgacccaagaaaccagaatccaaattcatttctgaacaactatattggctgttcttaacttccaagtacatatggttttcattcccaaggttcacatgtttaatagctactttgggttgatcagccacagattggacagaaacatcaggatgatgtattaatttataagtactaggttcattaatcttatttttcaggccaataacctcttccttccattggtctatttttttaaccgcttcctgaagttgttcagaatcaaaagttattttagaatcacctgatttactgtttttgtccttcagattaacatgtttttccttcaaaaaagctagttgaggttggtcagtcattgactgaggtggaacattagaatccaaaattatttcagaaccactacatttatcattcttgttttctagaacatattgcttctttctgtttattttgttaacagctacttgaggttcagttactgaataatgagggacaccagaatctaaacttgtttttgaaccactgaattcagtacttctaccttggaattcagcgtgcttttctctttgaagccatgtttctttgacaattacttcaggtttgtgagtcgctgcctgaagagggacatcagaatccaaacttgtttcaaaaacactcttattttctaagtacatgtgctcttttgtgtgaaggcttatttctttaatgggatcttcagaacgtccagtcactgaatgaaaaatgatattataatccaaacttacttcagaatcaataggttcattttccttattttctaagtgtacctgctcttctttttgaggatttagctttttaacagctacttcgggagaattagtcactgaatgaagaggggcatgggaatccgaacttatttcagaaccactgggttcatcattcttcctttctaagtgaatgtactcttctttctgaattacttctttaacagctacttcagggtgatcatttcctgaatgaagaggaatatcagaatcaaaagttatttcagagacacaagattcattacttttactttccagatcaacagtttcttcctcataaacagctacttcaggttggtcaattactgaataaagaggaatatcagaatcaaaagttatttcagaactatctgactcacagctctcatcttccaggtcaatgtgccgttcttttccttcagcatccagatgagactgctcagtaactgacagaagaggcgggtcagaatcaaaagtcaactcagagctggagcaatcatagctcctaacttccatgtcaatatttaactctttaagatttacttcatccaaagcttcttgaggctcatcatgagctgaatgataaagagaagccggagaatcagaactcagagaagaacggctagactgaacactcttattctcaaggtcaacatccactttctgacgctctatttcggctacttgagactggtcagctaattgagcatcagcctgaaaacccatttcaggaccatgggattcacagttcatatccataaggtcagcattcttctccttcagaagatttatcttttcaacagccctctgggattcatctgcaactgtcccaagtgagacatcacaatcaagatgtgctttagcactactgggtttacgcttcttatgttttaggtggacttgtctacctttcaggtttcttcctttgacagtcagttggggatgatcaactactgactcaagagaaacatcacaatcaaaacttgtttcagaacaactcgatccatagttatcaaccaagctggtatgagccttcttccgaagttttgtttctgtgacagccactgggggtctgtcaaccactgactgcagtgggaaaacagaatcagcacttacttcagagctactggaaccatagttcttatcaaccaaaccaatgtgcacttccttaggaaggtttacttctgttacagattgttgggggtagtcactagtggactgaggtgaagcatcacaatcaaaattcgtttcagaactactagattcatagctttggtcaaccaggctaatatgccttgcattctgaagacttatttctttaacaatcatttgggattggttggtaaccaagtgaagaatgtcatcacaatcagaacttattttagaaacataagatttattattcttatactgtacatcagtacgtacttccttggaaaggtttacttctttggcactcactttagattggtcagtcagtgaatgaaaagaggaactgcaatcaaaactcatttctgaacctctagactcatagttatcttcttggtcaatttgctcctccttccaaagacttaagtcttgtgcagtctcttggggctgatcagatgctgactgaagagagatacaatcaaacttcatttcagaactcactgagcacttctgttcccaaaaggctgtcttgttaaaaaccaaatgcttttcttcttgggtacaatccatgttagaaaagaattcctcatggttctttgcaatagtatcttcaaagattcctttattagaaggcatgtcagttttattcgggtttactgctaatttggaaggagatttaactcttaaggagcccttagtacccatgcgttcatggaatttcaagccagctgataaagttttaccctgagattttacatctttccacaaaaccaacttatctgaattcatgcgtaaagatttcctatttgattctttatgtttctgatacgaaaatgaagtagtttctacatgggatgatggcacaggatttctagaggccccatctggctgttcaagatatttctcaactttgtttgggtcacatttgctaactgaatccaaatgagctgctggtggtaaactagttgtattagctgtaactggtctatcgttagagctttcaggtaaacaactagcaggagcattacaaatcactggggggcgtaccaagttgcttctattatttgtagcctgaccaatatctactaggttacattttctcacactggccccaattttatgaacaaactccaagggctgctgctgtcccttctccagtttttgaataactgatggtcgaactgaaacctcctgcgtgccttcctgagatttatgaggtctggaatgtaactcttcaataggttctgaaacctcggatggtctctcttcggtagcatcctcatcctcaaccttatcctcatcctcttcctcttcttcagaaaaagcatcatccaaatgcaccacttcagacgatgacccagtattcacatgtgtctcatcttgtgttgaactgctctcttgacaatgatatgggtggtgctgcagtacatcctgtaagaaacgttccatcaaactactggtacatatttgacgtctactctgtctggtcaaactcctgtgctgagcactgaacaaatgctgttccaggttattatactgcacacggcaataactgcaatatccttgtcttttctgcatcttgaataaataactgaagtcagatggctactgtctttgaatactcaagctggagcagaaaaggtcaggtatttcatcagctgtattagttctggcaagtatctccgcggaggctgcccggattccttccgggccgcggtggagaccgaggaccgagccgggcgctctcccttcttattccggttccgcggcggcgcccgaatcccagaccgtccgagcgccacggccccgctgcccgcggagccagaaataggcgacttcggcccctgcggtccggaggcgagaagcggcgcgggagcgcgtctctcaggacgcgggccccgagtcgcgactccactcacgcaggcatccaaggcaacgtggcgttgcaaccctgatggaggttt

SEQ ID NO: 18367 - RNA, 8214 nt, Homo sapiens
  source 1..8214: mol_type = other RNA
tgaagtaccagctactcgagaggcttaggcaggagaattgcttgaacccgggaggtggaggttgcggtgagctaagttcaggccactgcactccagcctgggcaagacagtgagactctgtctcaaaaaataataataataaataaacataaaaataaaaactgatatggtaatgcctaaaatatttttaggggataaggccacaaaataacctggattttcatattaagccaccaactcttcatgtagaagagagtaaaggtggttaaaaaaaagggggggaatgcctaaacacatgggcaaaattattttcccctttaagatctaataaggctaacccaaaaaacctagagactgtatgtgtgcatgtgtccaaatgataaaagttagagacttgcagatccaatttaaatgaagcaggaggagtttgtgctatgcataaaaaaaatcaccagtttttaaaaactgtattaaagattatggaatctcattttctggaatgctttaaaaagaaagaaaacttatattttgtttgtattcatttaagtcaaccccattcaaaagttgacataattcattataattccttctttttaataagtttgctatattcattctcacaatgttaaatttgctggcatgagagagataatcataaaaaataagagggatatgatttgaggaacaaaattctatatacggtgctaaattattttgtgacataaattaagatgaagttcttctacagaaaatgttggacaaaggctgtttctgaatcttaaaatgaaaggactctaaacactaattttaaatgaatataaaaattctgaaaaataatatttatagcaaaatagttcaagattagttttctcaccaaagctgggaaagctgtgtgcacaaagtaccaaatatatttcaactgaagtactgaatcctcaactagcctgaacacaaaaccaacttctattttacctcattacctctcagtttgtttgctagccgagtcatcattctctcacgttgttgtaaacaagatgagcttctcagatcatatgctctcacaggtgtagaaggacctttctgtcggccatggtagctttcatcagtcttcttcctccttcttgcaacgcggcaagaagcccgcacaggtcgctttggaggaggatttgccatagcgcttgacagctcttcggcaccagctggtggaactgaagagttcaaaagcactttagctgttctcttcgccttctttagcctactgacaacagattttttcttcttcagataccttccaagaaaagcgctcctggactgatatctatgacgtaaaaagacagagtatttcgaaatatactttctaatgatatcacttggtttggtccgaatccaaattgactgtttctctgaagcttttctgggtttttgctggagaataattggtttataaacctttttgggaaaacctagcttattactactagttgtcaccctctttccatgaattttctttttactttgactttccaaaagcttatttctaactgattttggagagattttgacaacatcatgatttaaaaatgttagctggaaatttcttttctttggaagctcacgagcatgcagaacctttgattcttccagaaacagagaagagtcactggttccctgatgtgaattaaatccatatcttgccggcactgccattaaaggcgctgaagcagagccttgtccatcagcatcattatctcctgcactggagttttggttgctcctattaaaatgaattttaacccagttacgcctctcaaactctggtactattacactcaggggaggactaattacaatttgcttaatcaagggctcataataatcaaagatattccgtttatatttgcatataaaccgaatatcattatcccaactatggtgcctcattttagggaaaggaaggccttcaccctctttcagtttaatatttaaagaagaaagaacacagactaaggctttgggttgcataggcttcaaaactttagtacatgatgcaggaaattcaactgtcccaattttgactttctttttggtttttctgtcatcctgtaaacgtgaacacttactttttggtgggtcttcctcttgtctaattatttttcttttcatcactgggtaattcttacaactggtctgagtactatggctgattttcgctgtctggcattgagaagccacacgccccttttgcttaggaggcctctctgctggaggatgacgatggcatggtttatctaaggccactgacaagtcatcaatatctgaaataccacagacaatatcatcactctctgacacagcttgagttggtgcagtgtcctccttaccttgcaagtcagcccaggtaaccttttttttccccttcgaagaaacttttttggtctcacagtcatcatcaaagtaacagtggaaacgaccttccctaaactccttcaccagagcattaatttttatgtcatcttctctcattatctgagaccatgttttccccacaaatgaaggaggtacatgaggcaaggcttcaagaactggttcatcaggattatcctctatgacatcctttgcttttttcaggttccttacagaatcaaccttgagaacagagcttgactgggaatcatggttcttttctttcaagtcagaagataccttcttacaagggtgtcttttcttaacagtttcttgaggctgatcagtatcagatggaagagggggagcacactgaaaattcatctcaaaaccatccggttcacagctcacttctagatctctatgttttagcttcgaacgtttttttttatcagcccttcgatggagcgctgacttggaagaggcaccaaaatccactgcagaagcactagactgacagctcttaccttttaggccagcatttcttggatccttccgaagactggcttctttgtgagctttctgcagtcggtgagtcgttcgatgagaagtgtcttccaaattaaattttcctttagaaccattatatccacagctcttatcttctgaatcaatatatttcaccattttctcatcaggtccttgtgactcgtaagtcatggactgatcagaggcatcaacattaaaattcatttcagaaccacaagattgacaacttggctctcccagaataatatagtccttcttccggtttattattttgaaagtctctttgcattggtttgtcattgagggagtagaggctttacaattacatctgacttcagaaccaaaaaagtcacagctcttatcttctatatcaatacattctgtatttatacagctgatatctttgacagtcaactgaggtgggtcagtcactaactgaaggggaatatcatctgaaattacttcataatcactatcaccgggcaccagatccacaagtaccacctttggaaggtgggtttctttgactgatcctggaaattggttaactactatttgaaaaggaacatcagaatcatacatcatttctgaatcactaggttgatcggtcttttcttccatgacaacatgctcttccttctgaaggtctgcctctttgtaagacacttgaggttggtcaacttctgactgaagatgaacacaagaatgacattttatttcagaaccacagacttcacagttcttattttctagatcattatgatccttcttttgcaagtttatttctttgacaggtacagaagattgatcagtcacaaactgaacaggaatatgagaagcataacttacatcaaaatcacctaatttatagctcttatcttccaggtaaatatggtcttccttccaaagatttatttctttgacaggtttttgaagctcatctgctgctgcctgaaaagagtcattggaatcagaactttcttcaggactataagaattactgctcttatcttccagactggcatgctcctcttccaaaatgtgtggttgttttatcactgactgaagagggatatttgaaacataaattatttcagaatcactgggcacatagcccttatcatccagacaaacatgttcctccctcaaaagatttatttctttattcgcccctggaattttattagttacggactgaaggggttcatgagaatcaaaatttattctggaatctgtaggtttgacaatcttattttccaagtcaacatgctctttccaaagactgacctccttaactacttcttcaggttggccagccactggctgaagaacatcagaatcatacataatttcaaaacccttagcttcatttctcctatcttccgtgtcaacttcttcatccttccaaaggcttatttctttaacggtttctctcagccggtcagccactgactgaagagggtcatcagaatcaaaacttacttcagaaccacaacattgattgtgcttaccttctagttcaatgtgctcctgctccaaaatagttatttgaggtcgattgactattgactgacccaagaaaccagaatccaaattcatttctgaacaactatattggctgttcttaacttccaagtacatatggttttcattcccaaggttcacatgtttaatagctactttgggttgatcagccacagattggacagaaacatcaggatgatgtattaatttataagtactaggttcattaatcttatttttcaggccaataacctcttccttccattggtctatttttttaaccgcttcctgaagttgttcagaatcaaaagttattttagaatcacctgatttactgtttttgtccttcagattaacatgtttttccttcaaaaaagctagttgaggttggtcagtcattgactgaggtggaacattagaatccaaaattatttcagaaccactacatttatcattcttgttttctagaacatattgcttctttctgtttattttgttaacagctacttgaggttcagttactgaataatgagggacaccagaatctaaacttgtttttgaaccactgaattcagtacttctaccttggaattcagcgtgcttttctctttgaagccatgtttctttgacaattacttcaggtttgtgagtcgctgcctgaagagggacatcagaatccaaacttgtttcaaaaacactcttattttctaagtacatgtgctcttttgtgtgaaggcttatttctttaatgggatcttcagaacgtccagtcactgaatgaaaaatgatattataatccaaacttacttcagaatcaataggttcattttccttattttctaagtgtacctgctcttctttttgaggatttagctttttaacagctacttcgggagaattagtcactgaatgaagaggggcatgggaatccgaacttatttcagaaccactgggttcatcattcttcctttctaagtgaatgtactcttctttctgaattacttctttaacagctacttcagggtgatcatttcctgaatgaagaggaatatcagaatcaaaagttatttcagagacacaagattcattacttttactttccagatcaacagtttcttcctcataaacagctacttcaggttggtcaattactgaataaagaggaatatcagaatcaaaagttatttcagaactatctgactcacagctctcatcttccaggtcaatgtgccgttcttttccttcagcatccagatgagactgctcagtaactgacagaagaggcgggtcagaatcaaaagtcaactcagagctggagcaatcatagctcctaacttccatgtcaatatttaactctttaagatttacttcatccaaagcttcttgaggctcatcatgagctgaatgataaagagaagccggagaatcagaactcagagaagaacggctagactgaacactcttattctcaaggtcaacatccactttctgacgctctatttcggctacttgagactggtcagctaattgagcatcagcctgaaaacccatttcaggaccatgggattcacagttcatatccataaggtcagcattcttctccttcagaagatttatcttttcaacagccctctgggattcatctgcaactgtcccaagtgagacatcacaatcaagatgtgctttagcactactgggtttacgcttcttatgttttaggtggacttgtctacctttcaggtttcttcctttgacagtcagttggggatgatcaactactgactcaagagaaacatcacaatcaaaacttgtttcagaacaactcgatccatagttatcaaccaagctggtatgagccttcttccgaagttttgtttctgtgacagccactgggggtctgtcaaccactgactgcagtgggaaaacagaatcagcacttacttcagagctactggaaccatagttcttatcaaccaaaccaatgtgcacttccttaggaaggtttacttctgttacagattgttgggggtagtcactagtggactgaggtgaagcatcacaatcaaaattcgtttcagaactactagattcatagctttggtcaaccaggctaatatgccttgcattctgaagacttatttctttaacaatcatttgggattggttggtaaccaagtgaagaatgtcatcacaatcagaacttattttagaaacataagatttattattcttatactgtacatcagtacgtacttccttggaaaggtttacttctttggcactcactttagattggtcagtcagtgaatgaaaagaggaactgcaatcaaaactcatttctgaacctctagactcatagttatcttcttggtcaatttgctcctccttccaaagacttaagtcttgtgcagtctcttggggctgatcagatgctgactgaagagagatacaatcaaacttcatttcagaactcactgagcacttctgttcccaaaaggctgtcttgttaaaaaccaaatgcttttcttcttgggtacaatccatgttagaaaagaattcctcatggttctttgcaatagtatcttcaaagattcctttattagaaggcatgtcagttttattcgggtttactgctaatttggaaggagatttaactcttaaggagcccttagtacccatgcgttcatggaatttcaagccagctgataaagttttaccctgagattttacatctttccacaaaaccaacttatctgaattcatgcgtaaagatttcctatttgattctttatgtttctgatacgaaaatgaagtagtttctacatgggatgatggcacaggatttctagaggccccatctggctgttcaagatatttctcaactttgtttgggtcacatttgctaactgaatccaaatgagctgctggtggtaaactagttgtattagctgtaactggtctatcgttagagctttcaggtaaacaactagcaggagcattacaaatcactggggggcgtaccaagttgcttctattatttgtagcctgaccaatatctactaggttacattttctcacactggccccaattttatgaacaaactccaagggctgctgctgtcccttctccagtttttgaataactgatggtcgaactgaaacctcctgcgtgccttcctgagatttatgaggtctggaatgtaactcttcaataggttctgaaacctcggatggtctctcttcggtagcatcctcatcctcaaccttatcctcatcctcttcctcttcttcagaaaaagcatcatccaaatgcaccacttcagacgatgacccagtattcacatgtgtctcatcttgtgttgaactgctctcttgacaatgatatgggtggtgctgcagtacatcctgtaagaaacgttccatcaaactactggtacatatttgacgtctactctgtctggtcaaactcctgtgctgagcactgaacaaatgctgttccaggttattatactgcacacggcaataactgcaatatccttgtcttttctgcatcttgaataaataactgaagtcagatggctactgtctttgaatactcaagctggagcagaaaaggtcaggtatttcatcagctgtattagttctggcaagtatctccttccctcgccccgccacctcgatcccggcccggagccgccgacacctctcacgcagcaggggcagaaagggacgcggggt

SEQ ID NO: 18368 - RNA, 8209 nt, Homo sapiens
  source 1..8209: mol_type = other RNA
tgaagtaccagctactcgagaggcttaggcaggagaattgcttgaacccgggaggtggaggttgcggtgagctaagttcaggccactgcactccagcctgggcaagacagtgagactctgtctcaaaaaataataataataaataaacataaaaataaaaactgatatggtaatgcctaaaatatttttaggggataaggccacaaaataacctggattttcatattaagccaccaactcttcatgtagaagagagtaaaggtggttaaaaaaaagggggggaatgcctaaacacatgggcaaaattattttcccctttaagatctaataaggctaacccaaaaaacctagagactgtatgtgtgcatgtgtccaaatgataaaagttagagacttgcagatccaatttaaatgaagcaggaggagtttgtgctatgcataaaaaaaatcaccagtttttaaaaactgtattaaagattatggaatctcattttctggaatgctttaaaaagaaagaaaacttatattttgtttgtattcatttaagtcaaccccattcaaaagttgacataattcattataattccttctttttaataagtttgctatattcattctcacaatgttaaatttgctggcatgagagagataatcataaaaaataagagggatatgatttgaggaacaaaattctatatacggtgctaaattattttgtgacataaattaagatgaagttcttctacagaaaatgttggacaaaggctgtttctgaatcttaaaatgaaaggactctaaacactaattttaaatgaatataaaaattctgaaaaataatatttatagcaaaatagttcaagattagttttctcaccaaagctgggaaagctgtgtgcacaaagtaccaaatatatttcaactgaagtactgaatcctcaactagcctgaacacaaaaccaacttctattttacctcattacctctcagtttgtttgctagccgagtcatcattctctcacgttgttgtaaacaagatgagcttctcagatcatatgctctcacaggtgtagaaggacctttctgtcggccatggtagctttcatcagtcttcttcctccttcttgcaacgcggcaagaagcccgcacaggtcgctttggaggaggatttgccatagcgcttgacagctcttcggcaccagctggtggaactgaagagttcaaaagcactttagctgttctcttcgccttctttagcctactgacaacagattttttcttcttcagataccttccaagaaaagcgctcctggactgatatctatgacgtaaaaagacagagtatttcgaaatatactttctaatgatatcacttggtttggtccgaatccaaattgactgtttctctgaagcttttctgggtttttgctggagaataattggtttataaacctttttgggaaaacctagcttattactactagttgtcaccctctttccatgaattttctttttactttgactttccaaaagcttatttctaactgattttggagagattttgacaacatcatgatttaaaaatgttagctggaaatttcttttctttggaagctcacgagcatgcagaacctttgattcttccagaaacagagaagagtcactggttccctgatgtgaattaaatccatatcttgccggcactgccattaaaggcgctgaagcagagccttgtccatcagcatcattatctcctgcactggagttttggttgctcctattaaaatgaattttaacccagttacgcctctcaaactctggtactattacactcaggggaggactaattacaatttgcttaatcaagggctcataataatcaaagatattccgtttatatttgcatataaaccgaatatcattatcccaactatggtgcctcattttagggaaaggaaggccttcaccctctttcagtttaatatttaaagaagaaagaacacagactaaggctttgggttgcataggcttcaaaactttagtacatgatgcaggaaattcaactgtcccaattttgactttctttttggtttttctgtcatcctgtaaacgtgaacacttactttttggtgggtcttcctcttgtctaattatttttcttttcatcactgggtaattcttacaactggtctgagtactatggctgattttcgctgtctggcattgagaagccacacgccccttttgcttaggaggcctctctgctggaggatgacgatggcatggtttatctaaggccactgacaagtcatcaatatctgaaataccacagacaatatcatcactctctgacacagcttgagttggtgcagtgtcctccttaccttgcaagtcagcccaggtaaccttttttttccccttcgaagaaacttttttggtctcacagtcatcatcaaagtaacagtggaaacgaccttccctaaactccttcaccagagcattaatttttatgtcatcttctctcattatctgagaccatgttttccccacaaatgaaggaggtacatgaggcaaggcttcaagaactggttcatcaggattatcctctatgacatcctttgcttttttcaggttccttacagaatcaaccttgagaacagagcttgactgggaatcatggttcttttctttcaagtcagaagataccttcttacaagggtgtcttttcttaacagtttcttgaggctgatcagtatcagatggaagagggggagcacactgaaaattcatctcaaaaccatccggttcacagctcacttctagatctctatgttttagcttcgaacgtttttttttatcagcccttcgatggagcgctgacttggaagaggcaccaaaatccactgcagaagcactagactgacagctcttaccttttaggccagcatttcttggatccttccgaagactggcttctttgtgagctttctgcagtcggtgagtcgttcgatgagaagtgtcttccaaattaaattttcctttagaaccattatatccacagctcttatcttctgaatcaatatatttcaccattttctcatcaggtccttgtgactcgtaagtcatggactgatcagaggcatcaacattaaaattcatttcagaaccacaagattgacaacttggctctcccagaataatatagtccttcttccggtttattattttgaaagtctctttgcattggtttgtcattgagggagtagaggctttacaattacatctgacttcagaaccaaaaaagtcacagctcttatcttctatatcaatacattctgtatttatacagctgatatctttgacagtcaactgaggtgggtcagtcactaactgaaggggaatatcatctgaaattacttcataatcactatcaccgggcaccagatccacaagtaccacctttggaaggtgggtttctttgactgatcctggaaattggttaactactatttgaaaaggaacatcagaatcatacatcatttctgaatcactaggttgatcggtcttttcttccatgacaacatgctcttccttctgaaggtctgcctctttgtaagacacttgaggttggtcaacttctgactgaagatgaacacaagaatgacattttatttcagaaccacagacttcacagttcttattttctagatcattatgatccttcttttgcaagtttatttctttgacaggtacagaagattgatcagtcacaaactgaacaggaatatgagaagcataacttacatcaaaatcacctaatttatagctcttatcttccaggtaaatatggtcttccttccaaagatttatttctttgacaggtttttgaagctcatctgctgctgcctgaaaagagtcattggaatcagaactttcttcaggactataagaattactgctcttatcttccagactggcatgctcctcttccaaaatgtgtggttgttttatcactgactgaagagggatatttgaaacataaattatttcagaatcactgggcacatagcccttatcatccagacaaacatgttcctccctcaaaagatttatttctttattcgcccctggaattttattagttacggactgaaggggttcatgagaatcaaaatttattctggaatctgtaggtttgacaatcttattttccaagtcaacatgctctttccaaagactgacctccttaactacttcttcaggttggccagccactggctgaagaacatcagaatcatacataatttcaaaacccttagcttcatttctcctatcttccgtgtcaacttcttcatccttccaaaggcttatttctttaacggtttctctcagccggtcagccactgactgaagagggtcatcagaatcaaaacttacttcagaaccacaacattgattgtgcttaccttctagttcaatgtgctcctgctccaaaatagttatttgaggtcgattgactattgactgacccaagaaaccagaatccaaattcatttctgaacaactatattggctgttcttaacttccaagtacatatggttttcattcccaaggttcacatgtttaatagctactttgggttgatcagccacagattggacagaaacatcaggatgatgtattaatttataagtactaggttcattaatcttatttttcaggccaataacctcttccttccattggtctatttttttaaccgcttcctgaagttgttcagaatcaaaagttattttagaatcacctgatttactgtttttgtccttcagattaacatgtttttccttcaaaaaagctagttgaggttggtcagtcattgactgaggtggaacattagaatccaaaattatttcagaaccactacatttatcattcttgttttctagaacatattgcttctttctgtttattttgttaacagctacttgaggttcagttactgaataatgagggacaccagaatctaaacttgtttttgaaccactgaattcagtacttctaccttggaattcagcgtgcttttctctttgaagccatgtttctttgacaattacttcaggtttgtgagtcgctgcctgaagagggacatcagaatccaaacttgtttcaaaaacactcttattttctaagtacatgtgctcttttgtgtgaaggcttatttctttaatgggatcttcagaacgtccagtcactgaatgaaaaatgatattataatccaaacttacttcagaatcaataggttcattttccttattttctaagtgtacctgctcttctttttgaggatttagctttttaacagctacttcgggagaattagtcactgaatgaagaggggcatgggaatccgaacttatttcagaaccactgggttcatcattcttcctttctaagtgaatgtactcttctttctgaattacttctttaacagctacttcagggtgatcatttcctgaatgaagaggaatatcagaatcaaaagttatttcagagacacaagattcattacttttactttccagatcaacagtttcttcctcataaacagctacttcaggttggtcaattactgaataaagaggaatatcagaatcaaaagttatttcagaactatctgactcacagctctcatcttccaggtcaatgtgccgttcttttccttcagcatccagatgagactgctcagtaactgacagaagaggcgggtcagaatcaaaagtcaactcagagctggagcaatcatagctcctaacttccatgtcaatatttaactctttaagatttacttcatccaaagcttcttgaggctcatcatgagctgaatgataaagagaagccggagaatcagaactcagagaagaacggctagactgaacactcttattctcaaggtcaacatccactttctgacgctctatttcggctacttgagactggtcagctaattgagcatcagcctgaaaacccatttcaggaccatgggattcacagttcatatccataaggtcagcattcttctccttcagaagatttatcttttcaacagccctctgggattcatctgcaactgtcccaagtgagacatcacaatcaagatgtgctttagcactactgggtttacgcttcttatgttttaggtggacttgtctacctttcaggtttcttcctttgacagtcagttggggatgatcaactactgactcaagagaaacatcacaatcaaaacttgtttcagaacaactcgatccatagttatcaaccaagctggtatgagccttcttccgaagttttgtttctgtgacagccactgggggtctgtcaaccactgactgcagtgggaaaacagaatcagcacttacttcagagctactggaaccatagttcttatcaaccaaaccaatgtgcacttccttaggaaggtttacttctgttacagattgttgggggtagtcactagtggactgaggtgaagcatcacaatcaaaattcgtttcagaactactagattcatagctttggtcaaccaggctaatatgccttgcattctgaagacttatttctttaacaatcatttgggattggttggtaaccaagtgaagaatgtcatcacaatcagaacttattttagaaacataagatttattattcttatactgtacatcagtacgtacttccttggaaaggtttacttctttggcactcactttagattggtcagtcagtgaatgaaaagaggaactgcaatcaaaactcatttctgaacctctagactcatagttatcttcttggtcaatttgctcctccttccaaagacttaagtcttgtgcagtctcttggggctgatcagatgctgactgaagagagatacaatcaaacttcatttcagaactcactgagcacttctgttcccaaaaggctgtcttgttaaaaaccaaatgcttttcttcttgggtacaatccatgttagaaaagaattcctcatggttctttgcaatagtatcttcaaagattcctttattagaaggcatgtcagttttattcgggtttactgctaatttggaaggagatttaactcttaaggagcccttagtacccatgcgttcatggaatttcaagccagctgataaagttttaccctgagattttacatctttccacaaaaccaacttatctgaattcatgcgtaaagatttcctatttgattctttatgtttctgatacgaaaatgaagtagtttctacatgggatgatggcacaggatttctagaggccccatctggctgttcaagatatttctcaactttgtttgggtcacatttgctaactgaatccaaatgagctgctggtggtaaactagttgtattagctgtaactggtctatcgttagagctttcaggtaaacaactagcaggagcattacaaatcactggggggcgtaccaagttgcttctattatttgtagcctgaccaatatctactaggttacattttctcacactggccccaattttatgaacaaactccaagggctgctgctgtcccttctccagtttttgaataactgatggtcgaactgaaacctcctgcgtgccttcctgagatttatgaggtctggaatgtaactcttcaataggttctgaaacctcggatggtctctcttcggtagcatcctcatcctcaaccttatcctcatcctcttcctcttcttcagaaaaagcatcatccaaatgcaccacttcagacgatgacccagtattcacatgtgtctcatcttgtgttgaactgctctcttgacaatgatatgggtggtgctgcagtacatcctgtaagaaacgttccatcaaactactggtacatatttgacgtctactctgtctggtcaaactcctgtgctgagcactgaacaaatgctgttccaggttattatactgcacacggcaataactgcaatatccttgtcttttctgcatcttgaataaataactgaagtcagatggctactgtctttgaatactcaagctggagcagaaaaggtcaggtatttcatcagctgtattagttctggcaagtatctgcgaggcggccgcgggagcccagcgagcggtcctggcgtccctcgggaagaaggcgccccgggcgcccggcgagcag

SEQ ID NO: 18369 - RNA, 8458 nt, Homo sapiens
  source 1..8458: mol_type = other RNA
tgaagtaccagctactcgagaggcttaggcaggagaattgcttgaacccgggaggtggaggttgcggtgagctaagttcaggccactgcactccagcctgggcaagacagtgagactctgtctcaaaaaataataataataaataaacataaaaataaaaactgatatggtaatgcctaaaatatttttaggggataaggccacaaaataacctggattttcatattaagccaccaactcttcatgtagaagagagtaaaggtggttaaaaaaaagggggggaatgcctaaacacatgggcaaaattattttcccctttaagatctaataaggctaacccaaaaaacctagagactgtatgtgtgcatgtgtccaaatgataaaagttagagacttgcagatccaatttaaatgaagcaggaggagtttgtgctatgcataaaaaaaatcaccagtttttaaaaactgtattaaagattatggaatctcattttctggaatgctttaaaaagaaagaaaacttatattttgtttgtattcatttaagtcaaccccattcaaaagttgacataattcattataattccttctttttaataagtttgctatattcattctcacaatgttaaatttgctggcatgagagagataatcataaaaaataagagggatatgatttgaggaacaaaattctatatacggtgctaaattattttgtgacataaattaagatgaagttcttctacagaaaatgttggacaaaggctgtttctgaatcttaaaatgaaaggactctaaacactaattttaaatgaatataaaaattctgaaaaataatatttatagcaaaatagttcaagattagttttctcaccaaagctgggaaagctgtgtgcacaaagtaccaaatatatttcaactgaagtactgaatcctcaactagcctgaacacaaaaccaacttctattttacctcattacctctcagtttgtttgctagccgagtcatcattctctcacgttgttgtaaacaagatgagcttctcagatcatatgctctcacaggtgtagaaggacctttctgtcggccatggtagctttcatcagtcttcttcctccttcttgcaacgcggcaagaagcccgcacaggtcgctttggaggaggatttgccatagcgcttgacagctcttcggcaccagctggtggaactgaagagttcaaaagcactttagctgttctcttcgccttctttagcctactgacaacagattttttcttcttcagataccttccaagaaaagcgctcctggactgatatctatgacgtaaaaagacagagtatttcgaaatatactttctaatgatatcacttggtttggtccgaatccaaattgactgtttctctgaagcttttctgggtttttgctggagaataattggtttataaacctttttgggaaaacctagcttattactactagttgtcaccctctttccatgaattttctttttactttgactttccaaaagcttatttctaactgattttggagagattttgacaacatcatgatttaaaaatgttagctggaaatttcttttctttggaagctcacgagcatgcagaacctttgattcttccagaaacagagaagagtcactggttccctgatgtgaattaaatccatatcttgccggcactgccattaaaggcgctgaagcagagccttgtccatcagcatcattatctcctgcactggagttttggttgctcctattaaaatgaattttaacccagttacgcctctcaaactctggtactattacactcaggggaggactaattacaatttgcttaatcaagggctcataataatcaaagatattccgtttatatttgcatataaaccgaatatcattatcccaactatggtgcctcattttagggaaaggaaggccttcaccctctttcagtttaatatttaaagaagaaagaacacagactaaggctttgggttgcataggcttcaaaactttagtacatgatgcaggaaattcaactgtcccaattttgactttctttttggtttttctgtcatcctgtaaacgtgaacacttactttttggtgggtcttcctcttgtctaattatttttcttttcatcactgggtaattcttacaactggtctgagtactatggctgattttcgctgtctggcattgagaagccacacgccccttttgcttaggaggcctctctgctggaggatgacgatggcatggtttatctaaggccactgacaagtcatcaatatctgaaataccacagacaatatcatcactctctgacacagcttgagttggtgcagtgtcctccttaccttgcaagtcagcccaggtaaccttttttttccccttcgaagaaacttttttggtctcacagtcatcatcaaagtaacagtggaaacgaccttccctaaactccttcaccagagcattaatttttatgtcatcttctctcattatctgagaccatgttttccccacaaatgaaggaggtacatgaggcaaggcttcaagaactggttcatcaggattatcctctatgacatcctttgcttttttcaggttccttacagaatcaaccttgagaacagagcttgactgggaatcatggttcttttctttcaagtcagaagataccttcttacaagggtgtcttttcttaacagtttcttgaggctgatcagtatcagatggaagagggggagcacactgaaaattcatctcaaaaccatccggttcacagctcacttctagatctctatgttttagcttcgaacgtttttttttatcagcccttcgatggagcgctgacttggaagaggcaccaaaatccactgcagaagcactagactgacagctcttaccttttaggccagcatttcttggatccttccgaagactggcttctttgtgagctttctgcagtcggtgagtcgttcgatgagaagtgtcttccaaattaaattttcctttagaaccattatatccacagctcttatcttctgaatcaatatatttcaccattttctcatcaggtccttgtgactcgtaagtcatggactgatcagaggcatcaacattaaaattcatttcagaaccacaagattgacaacttggctctcccagaataatatagtccttcttccggtttattattttgaaagtctctttgcattggtttgtcattgagggagtagaggctttacaattacatctgacttcagaaccaaaaaagtcacagctcttatcttctatatcaatacattctgtatttatacagctgatatctttgacagtcaactgaggtgggtcagtcactaactgaaggggaatatcatctgaaattacttcataatcactatcaccgggcaccagatccacaagtaccacctttggaaggtgggtttctttgactgatcctggaaattggttaactactatttgaaaaggaacatcagaatcatacatcatttctgaatcactaggttgatcggtcttttcttccatgacaacatgctcttccttctgaaggtctgcctctttgtaagacacttgaggttggtcaacttctgactgaagatgaacacaagaatgacattttatttcagaaccacagacttcacagttcttattttctagatcattatgatccttcttttgcaagtttatttctttgacaggtacagaagattgatcagtcacaaactgaacaggaatatgagaagcataacttacatcaaaatcacctaatttatagctcttatcttccaggtaaatatggtcttccttccaaagatttatttctttgacaggtttttgaagctcatctgctgctgcctgaaaagagtcattggaatcagaactttcttcaggactataagaattactgctcttatcttccagactggcatgctcctcttccaaaatgtgtggttgttttatcactgactgaagagggatatttgaaacataaattatttcagaatcactgggcacatagcccttatcatccagacaaacatgttcctccctcaaaagatttatttctttattcgcccctggaattttattagttacggactgaaggggttcatgagaatcaaaatttattctggaatctgtaggtttgacaatcttattttccaagtcaacatgctctttccaaagactgacctccttaactacttcttcaggttggccagccactggctgaagaacatcagaatcatacataatttcaaaacccttagcttcatttctcctatcttccgtgtcaacttcttcatccttccaaaggcttatttctttaacggtttctctcagccggtcagccactgactgaagagggtcatcagaatcaaaacttacttcagaaccacaacattgattgtgcttaccttctagttcaatgtgctcctgctccaaaatagttatttgaggtcgattgactattgactgacccaagaaaccagaatccaaattcatttctgaacaactatattggctgttcttaacttccaagtacatatggttttcattcccaaggttcacatgtttaatagctactttgggttgatcagccacagattggacagaaacatcaggatgatgtattaatttataagtactaggttcattaatcttatttttcaggccaataacctcttccttccattggtctatttttttaaccgcttcctgaagttgttcagaatcaaaagttattttagaatcacctgatttactgtttttgtccttcagattaacatgtttttccttcaaaaaagctagttgaggttggtcagtcattgactgaggtggaacattagaatccaaaattatttcagaaccactacatttatcattcttgttttctagaacatattgcttctttctgtttattttgttaacagctacttgaggttcagttactgaataatgagggacaccagaatctaaacttgtttttgaaccactgaattcagtacttctaccttggaattcagcgtgcttttctctttgaagccatgtttctttgacaattacttcaggtttgtgagtcgctgcctgaagagggacatcagaatccaaacttgtttcaaaaacactcttattttctaagtacatgtgctcttttgtgtgaaggcttatttctttaatgggatcttcagaacgtccagtcactgaatgaaaaatgatattataatccaaacttacttcagaatcaataggttcattttccttattttctaagtgtacctgctcttctttttgaggatttagctttttaacagctacttcgggagaattagtcactgaatgaagaggggcatgggaatccgaacttatttcagaaccactgggttcatcattcttcctttctaagtgaatgtactcttctttctgaattacttctttaacagctacttcagggtgatcatttcctgaatgaagaggaatatcagaatcaaaagttatttcagagacacaagattcattacttttactttccagatcaacagtttcttcctcataaacagctacttcaggttggtcaattactgaataaagaggaatatcagaatcaaaagttatttcagaactatctgactcacagctctcatcttccaggtcaatgtgccgttcttttccttcagcatccagatgagactgctcagtaactgacagaagaggcgggtcagaatcaaaagtcaactcagagctggagcaatcatagctcctaacttccatgtcaatatttaactctttaagatttacttcatccaaagcttcttgaggctcatcatgagctgaatgataaagagaagccggagaatcagaactcagagaagaacggctagactgaacactcttattctcaaggtcaacatccactttctgacgctctatttcggctacttgagactggtcagctaattgagcatcagcctgaaaacccatttcaggaccatgggattcacagttcatatccataaggtcagcattcttctccttcagaagatttatcttttcaacagccctctgggattcatctgcaactgtcccaagtgagacatcacaatcaagatgtgctttagcactactgggtttacgcttcttatgttttaggtggacttgtctacctttcaggtttcttcctttgacagtcagttggggatgatcaactactgactcaagagaaacatcacaatcaaaacttgtttcagaacaactcgatccatagttatcaaccaagctggtatgagccttcttccgaagttttgtttctgtgacagccactgggggtctgtcaaccactgactgcagtgggaaaacagaatcagcacttacttcagagctactggaaccatagttcttatcaaccaaaccaatgtgcacttccttaggaaggtttacttctgttacagattgttgggggtagtcactagtggactgaggtgaagcatcacaatcaaaattcgtttcagaactactagattcatagctttggtcaaccaggctaatatgccttgcattctgaagacttatttctttaacaatcatttgggattggttggtaaccaagtgaagaatgtcatcacaatcagaacttattttagaaacataagatttattattcttatactgtacatcagtacgtacttccttggaaaggtttacttctttggcactcactttagattggtcagtcagtgaatgaaaagaggaactgcaatcaaaactcatttctgaacctctagactcatagttatcttcttggtcaatttgctcctccttccaaagacttaagtcttgtgcagtctcttggggctgatcagatgctgactgaagagagatacaatcaaacttcatttcagaactcactgagcacttctgttcccaaaaggctgtcttgttaaaaaccaaatgcttttcttcttgggtacaatccatgttagaaaagaattcctcatggttctttgcaatagtatcttcaaagattcctttattagaaggcatgtcagttttattcgggtttactgctaatttggaaggagatttaactcttaaggagcccttagtacccatgcgttcatggaatttcaagccagctgataaagttttaccctgagattttacatctttccacaaaaccaacttatctgaattcatgcgtaaagatttcctatttgattctttatgtttctgatacgaaaatgaagtagtttctacatgggatgatggcacaggatttctagaggccccatctggctgttcaagatatttctcaactttgtttgggtcacatttgctaactgaatccaaatgagctgctggtggtaaactagttgtattagctgtaactggtctatcgttagagctttcaggtaaacaactagcaggagcattacaaatcactggggggcgtaccaagttgcttctattatttgtagcctgaccaatatctactaggttacattttctcacactggccccaattttatgaacaaactccaagggctgctgctgtcccttctccagtttttgaataactgatggtcgaactgaaacctcctgcgtgccttcctgagatttatgaggtctggaatgtaactcttcaataggttctgaaacctcggatggtctctcttcggtagcatcctcatcctcaaccttatcctcatcctcttcctcttcttcagaaaaagcatcatccaaatgcaccacttcagacgatgacccagtattcacatgtgtctcatcttgtgttgaactgctctcttgacaatgatatgggtggtgctgcagtacatcctgtaagaaacgttccatcaaactactggtacatatttgacgtctactctgtctggtcaaactcctgtgctgagcactgaacaaatgctgttccaggttattatactgcacacggcaataactgcaatatccttgtcttttctgcatcttgaataaataactgaagtcagatggctactgtctttgaatactcaagttaaaatttggtctcttttccactaatttacttcacttattaacctggagcagaaaaggtcaggtatttcatcagctgtattagttctggcaagtatctccgcggaggctgcccggattccttccgggccgcggtggagaccgaggaccgagccgggcgctctcccttcttattccggttccgcggcggcgcccgaatcccagaccgtccgagcgccacggccccgctgcccgcggagccagaaataggcgacttcggcccctgcggtccggaggcgagaagcggcgcgggagcgcgtctctcaggacgcgggccccgagtcgcgactccactcacgcaggcatccaaggcaacgtggcgttgcaaccctgatggaggttt

SEQ ID NO: 18370 - RNA, 8258 nt, Homo sapiens
  source 1..8258: mol_type = other RNA
tgaagtaccagctactcgagaggcttaggcaggagaattgcttgaacccgggaggtggaggttgcggtgagctaagttcaggccactgcactccagcctgggcaagacagtgagactctgtctcaaaaaataataataataaataaacataaaaataaaaactgatatggtaatgcctaaaatatttttaggggataaggccacaaaataacctggattttcatattaagccaccaactcttcatgtagaagagagtaaaggtggttaaaaaaaagggggggaatgcctaaacacatgggcaaaattattttcccctttaagatctaataaggctaacccaaaaaacctagagactgtatgtgtgcatgtgtccaaatgataaaagttagagacttgcagatccaatttaaatgaagcaggaggagtttgtgctatgcataaaaaaaatcaccagtttttaaaaactgtattaaagattatggaatctcattttctggaatgctttaaaaagaaagaaaacttatattttgtttgtattcatttaagtcaaccccattcaaaagttgacataattcattataattccttctttttaataagtttgctatattcattctcacaatgttaaatttgctggcatgagagagataatcataaaaaataagagggatatgatttgaggaacaaaattctatatacggtgctaaattattttgtgacataaattaagatgaagttcttctacagaaaatgttggacaaaggctgtttctgaatcttaaaatgaaaggactctaaacactaattttaaatgaatataaaaattctgaaaaataatatttatagcaaaatagttcaagattagttttctcaccaaagctgggaaagctgtgtgcacaaagtaccaaatatatttcaactgaagtactgaatcctcaactagcctgaacacaaaaccaacttctattttacctcattacctctcagtttgtttgctagccgagtcatcattctctcacgttgttgtaaacaagatgagcttctcagatcatatgctctcacaggtgtagaaggacctttctgtcggccatggtagctttcatcagtcttcttcctccttcttgcaacgcggcaagaagcccgcacaggtcgctttggaggaggatttgccatagcgcttgacagctcttcggcaccagctggtggaactgaagagttcaaaagcactttagctgttctcttcgccttctttagcctactgacaacagattttttcttcttcagataccttccaagaaaagcgctcctggactgatatctatgacgtaaaaagacagagtatttcgaaatatactttctaatgatatcacttggtttggtccgaatccaaattgactgtttctctgaagcttttctgggtttttgctggagaataattggtttataaacctttttgggaaaacctagcttattactactagttgtcaccctctttccatgaattttctttttactttgactttccaaaagcttatttctaactgattttggagagattttgacaacatcatgatttaaaaatgttagctggaaatttcttttctttggaagctcacgagcatgcagaacctttgattcttccagaaacagagaagagtcactggttccctgatgtgaattaaatccatatcttgccggcactgccattaaaggcgctgaagcagagccttgtccatcagcatcattatctcctgcactggagttttggttgctcctattaaaatgaattttaacccagttacgcctctcaaactctggtactattacactcaggggaggactaattacaatttgcttaatcaagggctcataataatcaaagatattccgtttatatttgcatataaaccgaatatcattatcccaactatggtgcctcattttagggaaaggaaggccttcaccctctttcagtttaatatttaaagaagaaagaacacagactaaggctttgggttgcataggcttcaaaactttagtacatgatgcaggaaattcaactgtcccaattttgactttctttttggtttttctgtcatcctgtaaacgtgaacacttactttttggtgggtcttcctcttgtctaattatttttcttttcatcactgggtaattcttacaactggtctgagtactatggctgattttcgctgtctggcattgagaagccacacgccccttttgcttaggaggcctctctgctggaggatgacgatggcatggtttatctaaggccactgacaagtcatcaatatctgaaataccacagacaatatcatcactctctgacacagcttgagttggtgcagtgtcctccttaccttgcaagtcagcccaggtaaccttttttttccccttcgaagaaacttttttggtctcacagtcatcatcaaagtaacagtggaaacgaccttccctaaactccttcaccagagcattaatttttatgtcatcttctctcattatctgagaccatgttttccccacaaatgaaggaggtacatgaggcaaggcttcaagaactggttcatcaggattatcctctatgacatcctttgcttttttcaggttccttacagaatcaaccttgagaacagagcttgactgggaatcatggttcttttctttcaagtcagaagataccttcttacaagggtgtcttttcttaacagtttcttgaggctgatcagtatcagatggaagagggggagcacactgaaaattcatctcaaaaccatccggttcacagctcacttctagatctctatgttttagcttcgaacgtttttttttatcagcccttcgatggagcgctgacttggaagaggcaccaaaatccactgcagaagcactagactgacagctcttaccttttaggccagcatttcttggatccttccgaagactggcttctttgtgagctttctgcagtcggtgagtcgttcgatgagaagtgtcttccaaattaaattttcctttagaaccattatatccacagctcttatcttctgaatcaatatatttcaccattttctcatcaggtccttgtgactcgtaagtcatggactgatcagaggcatcaacattaaaattcatttcagaaccacaagattgacaacttggctctcccagaataatatagtccttcttccggtttattattttgaaagtctctttgcattggtttgtcattgagggagtagaggctttacaattacatctgacttcagaaccaaaaaagtcacagctcttatcttctatatcaatacattctgtatttatacagctgatatctttgacagtcaactgaggtgggtcagtcactaactgaaggggaatatcatctgaaattacttcataatcactatcaccgggcaccagatccacaagtaccacctttggaaggtgggtttctttgactgatcctggaaattggttaactactatttgaaaaggaacatcagaatcatacatcatttctgaatcactaggttgatcggtcttttcttccatgacaacatgctcttccttctgaaggtctgcctctttgtaagacacttgaggttggtcaacttctgactgaagatgaacacaagaatgacattttatttcagaaccacagacttcacagttcttattttctagatcattatgatccttcttttgcaagtttatttctttgacaggtacagaagattgatcagtcacaaactgaacaggaatatgagaagcataacttacatcaaaatcacctaatttatagctcttatcttccaggtaaatatggtcttccttccaaagatttatttctttgacaggtttttgaagctcatctgctgctgcctgaaaagagtcattggaatcagaactttcttcaggactataagaattactgctcttatcttccagactggcatgctcctcttccaaaatgtgtggttgttttatcactgactgaagagggatatttgaaacataaattatttcagaatcactgggcacatagcccttatcatccagacaaacatgttcctccctcaaaagatttatttctttattcgcccctggaattttattagttacggactgaaggggttcatgagaatcaaaatttattctggaatctgtaggtttgacaatcttattttccaagtcaacatgctctttccaaagactgacctccttaactacttcttcaggttggccagccactggctgaagaacatcagaatcatacataatttcaaaacccttagcttcatttctcctatcttccgtgtcaacttcttcatccttccaaaggcttatttctttaacggtttctctcagccggtcagccactgactgaagagggtcatcagaatcaaaacttacttcagaaccacaacattgattgtgcttaccttctagttcaatgtgctcctgctccaaaatagttatttgaggtcgattgactattgactgacccaagaaaccagaatccaaattcatttctgaacaactatattggctgttcttaacttccaagtacatatggttttcattcccaaggttcacatgtttaatagctactttgggttgatcagccacagattggacagaaacatcaggatgatgtattaatttataagtactaggttcattaatcttatttttcaggccaataacctcttccttccattggtctatttttttaaccgcttcctgaagttgttcagaatcaaaagttattttagaatcacctgatttactgtttttgtccttcagattaacatgtttttccttcaaaaaagctagttgaggttggtcagtcattgactgaggtggaacattagaatccaaaattatttcagaaccactacatttatcattcttgttttctagaacatattgcttctttctgtttattttgttaacagctacttgaggttcagttactgaataatgagggacaccagaatctaaacttgtttttgaaccactgaattcagtacttctaccttggaattcagcgtgcttttctctttgaagccatgtttctttgacaattacttcaggtttgtgagtcgctgcctgaagagggacatcagaatccaaacttgtttcaaaaacactcttattttctaagtacatgtgctcttttgtgtgaaggcttatttctttaatgggatcttcagaacgtccagtcactgaatgaaaaatgatattataatccaaacttacttcagaatcaataggttcattttccttattttctaagtgtacctgctcttctttttgaggatttagctttttaacagctacttcgggagaattagtcactgaatgaagaggggcatgggaatccgaacttatttcagaaccactgggttcatcattcttcctttctaagtgaatgtactcttctttctgaattacttctttaacagctacttcagggtgatcatttcctgaatgaagaggaatatcagaatcaaaagttatttcagagacacaagattcattacttttactttccagatcaacagtttcttcctcataaacagctacttcaggttggtcaattactgaataaagaggaatatcagaatcaaaagttatttcagaactatctgactcacagctctcatcttccaggtcaatgtgccgttcttttccttcagcatccagatgagactgctcagtaactgacagaagaggcgggtcagaatcaaaagtcaactcagagctggagcaatcatagctcctaacttccatgtcaatatttaactctttaagatttacttcatccaaagcttcttgaggctcatcatgagctgaatgataaagagaagccggagaatcagaactcagagaagaacggctagactgaacactcttattctcaaggtcaacatccactttctgacgctctatttcggctacttgagactggtcagctaattgagcatcagcctgaaaacccatttcaggaccatgggattcacagttcatatccataaggtcagcattcttctccttcagaagatttatcttttcaacagccctctgggattcatctgcaactgtcccaagtgagacatcacaatcaagatgtgctttagcactactgggtttacgcttcttatgttttaggtggacttgtctacctttcaggtttcttcctttgacagtcagttggggatgatcaactactgactcaagagaaacatcacaatcaaaacttgtttcagaacaactcgatccatagttatcaaccaagctggtatgagccttcttccgaagttttgtttctgtgacagccactgggggtctgtcaaccactgactgcagtgggaaaacagaatcagcacttacttcagagctactggaaccatagttcttatcaaccaaaccaatgtgcacttccttaggaaggtttacttctgttacagattgttgggggtagtcactagtggactgaggtgaagcatcacaatcaaaattcgtttcagaactactagattcatagctttggtcaaccaggctaatatgccttgcattctgaagacttatttctttaacaatcatttgggattggttggtaaccaagtgaagaatgtcatcacaatcagaacttattttagaaacataagatttattattcttatactgtacatcagtacgtacttccttggaaaggtttacttctttggcactcactttagattggtcagtcagtgaatgaaaagaggaactgcaatcaaaactcatttctgaacctctagactcatagttatcttcttggtcaatttgctcctccttccaaagacttaagtcttgtgcagtctcttggggctgatcagatgctgactgaagagagatacaatcaaacttcatttcagaactcactgagcacttctgttcccaaaaggctgtcttgttaaaaaccaaatgcttttcttcttgggtacaatccatgttagaaaagaattcctcatggttctttgcaatagtatcttcaaagattcctttattagaaggcatgtcagttttattcgggtttactgctaatttggaaggagatttaactcttaaggagcccttagtacccatgcgttcatggaatttcaagccagctgataaagttttaccctgagattttacatctttccacaaaaccaacttatctgaattcatgcgtaaagatttcctatttgattctttatgtttctgatacgaaaatgaagtagtttctacatgggatgatggcacaggatttctagaggccccatctggctgttcaagatatttctcaactttgtttgggtcacatttgctaactgaatccaaatgagctgctggtggtaaactagttgtattagctgtaactggtctatcgttagagctttcaggtaaacaactagcaggagcattacaaatcactggggggcgtaccaagttgcttctattatttgtagcctgaccaatatctactaggttacattttctcacactggccccaattttatgaacaaactccaagggctgctgctgtcccttctccagtttttgaataactgatggtcgaactgaaacctcctgcgtgccttcctgagatttatgaggtctggaatgtaactcttcaataggttctgaaacctcggatggtctctcttcggtagcatcctcatcctcaaccttatcctcatcctcttcctcttcttcagaaaaagcatcatccaaatgcaccacttcagacgatgacccagtattcacatgtgtctcatcttgtgttgaactgctctcttgacaatgatatgggtggtgctgcagtacatcctgtaagaaacgttccatcaaactactggtacatatttgacgtctactctgtctggtcaaactcctgtgctgagcactgaacaaatgctgttccaggttattatactgcacacggcaataactgcaatatccttgtcttttctgcatcttgaataaataactgaagtcagatggctactgtctttgaatactcaagttaaaatttggtctcttttccactaatttacttcacttattaacctggagcagaaaaggtcaggtatttcatcagctgtattagttctggcaagtatctccttccctcgccccgccacctcgatcccggcccggagccgccgacacctctcacgcagcaggggcagaaagggacgcggggt

SEQ ID NO: 18371 - RNA, 8253 nt, Homo sapiens
  source 1..8253: mol_type = other RNA
tgaagtaccagctactcgagaggcttaggcaggagaattgcttgaacccgggaggtggaggttgcggtgagctaagttcaggccactgcactccagcctgggcaagacagtgagactctgtctcaaaaaataataataataaataaacataaaaataaaaactgatatggtaatgcctaaaatatttttaggggataaggccacaaaataacctggattttcatattaagccaccaactcttcatgtagaagagagtaaaggtggttaaaaaaaagggggggaatgcctaaacacatgggcaaaattattttcccctttaagatctaataaggctaacccaaaaaacctagagactgtatgtgtgcatgtgtccaaatgataaaagttagagacttgcagatccaatttaaatgaagcaggaggagtttgtgctatgcataaaaaaaatcaccagtttttaaaaactgtattaaagattatggaatctcattttctggaatgctttaaaaagaaagaaaacttatattttgtttgtattcatttaagtcaaccccattcaaaagttgacataattcattataattccttctttttaataagtttgctatattcattctcacaatgttaaatttgctggcatgagagagataatcataaaaaataagagggatatgatttgaggaacaaaattctatatacggtgctaaattattttgtgacataaattaagatgaagttcttctacagaaaatgttggacaaaggctgtttctgaatcttaaaatgaaaggactctaaacactaattttaaatgaatataaaaattctgaaaaataatatttatagcaaaatagttcaagattagttttctcaccaaagctgggaaagctgtgtgcacaaagtaccaaatatatttcaactgaagtactgaatcctcaactagcctgaacacaaaaccaacttctattttacctcattacctctcagtttgtttgctagccgagtcatcattctctcacgttgttgtaaacaagatgagcttctcagatcatatgctctcacaggtgtagaaggacctttctgtcggccatggtagctttcatcagtcttcttcctccttcttgcaacgcggcaagaagcccgcacaggtcgctttggaggaggatttgccatagcgcttgacagctcttcggcaccagctggtggaactgaagagttcaaaagcactttagctgttctcttcgccttctttagcctactgacaacagattttttcttcttcagataccttccaagaaaagcgctcctggactgatatctatgacgtaaaaagacagagtatttcgaaatatactttctaatgatatcacttggtttggtccgaatccaaattgactgtttctctgaagcttttctgggtttttgctggagaataattggtttataaacctttttgggaaaacctagcttattactactagttgtcaccctctttccatgaattttctttttactttgactttccaaaagcttatttctaactgattttggagagattttgacaacatcatgatttaaaaatgttagctggaaatttcttttctttggaagctcacgagcatgcagaacctttgattcttccagaaacagagaagagtcactggttccctgatgtgaattaaatccatatcttgccggcactgccattaaaggcgctgaagcagagccttgtccatcagcatcattatctcctgcactggagttttggttgctcctattaaaatgaattttaacccagttacgcctctcaaactctggtactattacactcaggggaggactaattacaatttgcttaatcaagggctcataataatcaaagatattccgtttatatttgcatataaaccgaatatcattatcccaactatggtgcctcattttagggaaaggaaggccttcaccctctttcagtttaatatttaaagaagaaagaacacagactaaggctttgggttgcataggcttcaaaactttagtacatgatgcaggaaattcaactgtcccaattttgactttctttttggtttttctgtcatcctgtaaacgtgaacacttactttttggtgggtcttcctcttgtctaattatttttcttttcatcactgggtaattcttacaactggtctgagtactatggctgattttcgctgtctggcattgagaagccacacgccccttttgcttaggaggcctctctgctggaggatgacgatggcatggtttatctaaggccactgacaagtcatcaatatctgaaataccacagacaatatcatcactctctgacacagcttgagttggtgcagtgtcctccttaccttgcaagtcagcccaggtaaccttttttttccccttcgaagaaacttttttggtctcacagtcatcatcaaagtaacagtggaaacgaccttccctaaactccttcaccagagcattaatttttatgtcatcttctctcattatctgagaccatgttttccccacaaatgaaggaggtacatgaggcaaggcttcaagaactggttcatcaggattatcctctatgacatcctttgcttttttcaggttccttacagaatcaaccttgagaacagagcttgactgggaatcatggttcttttctttcaagtcagaagataccttcttacaagggtgtcttttcttaacagtttcttgaggctgatcagtatcagatggaagagggggagcacactgaaaattcatctcaaaaccatccggttcacagctcacttctagatctctatgttttagcttcgaacgtttttttttatcagcccttcgatggagcgctgacttggaagaggcaccaaaatccactgcagaagcactagactgacagctcttaccttttaggccagcatttcttggatccttccgaagactggcttctttgtgagctttctgcagtcggtgagtcgttcgatgagaagtgtcttccaaattaaattttcctttagaaccattatatccacagctcttatcttctgaatcaatatatttcaccattttctcatcaggtccttgtgactcgtaagtcatggactgatcagaggcatcaacattaaaattcatttcagaaccacaagattgacaacttggctctcccagaataatatagtccttcttccggtttattattttgaaagtctctttgcattggtttgtcattgagggagtagaggctttacaattacatctgacttcagaaccaaaaaagtcacagctcttatcttctatatcaatacattctgtatttatacagctgatatctttgacagtcaactgaggtgggtcagtcactaactgaaggggaatatcatctgaaattacttcataatcactatcaccgggcaccagatccacaagtaccacctttggaaggtgggtttctttgactgatcctggaaattggttaactactatttgaaaaggaacatcagaatcatacatcatttctgaatcactaggttgatcggtcttttcttccatgacaacatgctcttccttctgaaggtctgcctctttgtaagacacttgaggttggtcaacttctgactgaagatgaacacaagaatgacattttatttcagaaccacagacttcacagttcttattttctagatcattatgatccttcttttgcaagtttatttctttgacaggtacagaagattgatcagtcacaaactgaacaggaatatgagaagcataacttacatcaaaatcacctaatttatagctcttatcttccaggtaaatatggtcttccttccaaagatttatttctttgacaggtttttgaagctcatctgctgctgcctgaaaagagtcattggaatcagaactttcttcaggactataagaattactgctcttatcttccagactggcatgctcctcttccaaaatgtgtggttgttttatcactgactgaagagggatatttgaaacataaattatttcagaatcactgggcacatagcccttatcatccagacaaacatgttcctccctcaaaagatttatttctttattcgcccctggaattttattagttacggactgaaggggttcatgagaatcaaaatttattctggaatctgtaggtttgacaatcttattttccaagtcaacatgctctttccaaagactgacctccttaactacttcttcaggttggccagccactggctgaagaacatcagaatcatacataatttcaaaacccttagcttcatttctcctatcttccgtgtcaacttcttcatccttccaaaggcttatttctttaacggtttctctcagccggtcagccactgactgaagagggtcatcagaatcaaaacttacttcagaaccacaacattgattgtgcttaccttctagttcaatgtgctcctgctccaaaatagttatttgaggtcgattgactattgactgacccaagaaaccagaatccaaattcatttctgaacaactatattggctgttcttaacttccaagtacatatggttttcattcccaaggttcacatgtttaatagctactttgggttgatcagccacagattggacagaaacatcaggatgatgtattaatttataagtactaggttcattaatcttatttttcaggccaataacctcttccttccattggtctatttttttaaccgcttcctgaagttgttcagaatcaaaagttattttagaatcacctgatttactgtttttgtccttcagattaacatgtttttccttcaaaaaagctagttgaggttggtcagtcattgactgaggtggaacattagaatccaaaattatttcagaaccactacatttatcattcttgttttctagaacatattgcttctttctgtttattttgttaacagctacttgaggttcagttactgaataatgagggacaccagaatctaaacttgtttttgaaccactgaattcagtacttctaccttggaattcagcgtgcttttctctttgaagccatgtttctttgacaattacttcaggtttgtgagtcgctgcctgaagagggacatcagaatccaaacttgtttcaaaaacactcttattttctaagtacatgtgctcttttgtgtgaaggcttatttctttaatgggatcttcagaacgtccagtcactgaatgaaaaatgatattataatccaaacttacttcagaatcaataggttcattttccttattttctaagtgtacctgctcttctttttgaggatttagctttttaacagctacttcgggagaattagtcactgaatgaagaggggcatgggaatccgaacttatttcagaaccactgggttcatcattcttcctttctaagtgaatgtactcttctttctgaattacttctttaacagctacttcagggtgatcatttcctgaatgaagaggaatatcagaatcaaaagttatttcagagacacaagattcattacttttactttccagatcaacagtttcttcctcataaacagctacttcaggttggtcaattactgaataaagaggaatatcagaatcaaaagttatttcagaactatctgactcacagctctcatcttccaggtcaatgtgccgttcttttccttcagcatccagatgagactgctcagtaactgacagaagaggcgggtcagaatcaaaagtcaactcagagctggagcaatcatagctcctaacttccatgtcaatatttaactctttaagatttacttcatccaaagcttcttgaggctcatcatgagctgaatgataaagagaagccggagaatcagaactcagagaagaacggctagactgaacactcttattctcaaggtcaacatccactttctgacgctctatttcggctacttgagactggtcagctaattgagcatcagcctgaaaacccatttcaggaccatgggattcacagttcatatccataaggtcagcattcttctccttcagaagatttatcttttcaacagccctctgggattcatctgcaactgtcccaagtgagacatcacaatcaagatgtgctttagcactactgggtttacgcttcttatgttttaggtggacttgtctacctttcaggtttcttcctttgacagtcagttggggatgatcaactactgactcaagagaaacatcacaatcaaaacttgtttcagaacaactcgatccatagttatcaaccaagctggtatgagccttcttccgaagttttgtttctgtgacagccactgggggtctgtcaaccactgactgcagtgggaaaacagaatcagcacttacttcagagctactggaaccatagttcttatcaaccaaaccaatgtgcacttccttaggaaggtttacttctgttacagattgttgggggtagtcactagtggactgaggtgaagcatcacaatcaaaattcgtttcagaactactagattcatagctttggtcaaccaggctaatatgccttgcattctgaagacttatttctttaacaatcatttgggattggttggtaaccaagtgaagaatgtcatcacaatcagaacttattttagaaacataagatttattattcttatactgtacatcagtacgtacttccttggaaaggtttacttctttggcactcactttagattggtcagtcagtgaatgaaaagaggaactgcaatcaaaactcatttctgaacctctagactcatagttatcttcttggtcaatttgctcctccttccaaagacttaagtcttgtgcagtctcttggggctgatcagatgctgactgaagagagatacaatcaaacttcatttcagaactcactgagcacttctgttcccaaaaggctgtcttgttaaaaaccaaatgcttttcttcttgggtacaatccatgttagaaaagaattcctcatggttctttgcaatagtatcttcaaagattcctttattagaaggcatgtcagttttattcgggtttactgctaatttggaaggagatttaactcttaaggagcccttagtacccatgcgttcatggaatttcaagccagctgataaagttttaccctgagattttacatctttccacaaaaccaacttatctgaattcatgcgtaaagatttcctatttgattctttatgtttctgatacgaaaatgaagtagtttctacatgggatgatggcacaggatttctagaggccccatctggctgttcaagatatttctcaactttgtttgggtcacatttgctaactgaatccaaatgagctgctggtggtaaactagttgtattagctgtaactggtctatcgttagagctttcaggtaaacaactagcaggagcattacaaatcactggggggcgtaccaagttgcttctattatttgtagcctgaccaatatctactaggttacattttctcacactggccccaattttatgaacaaactccaagggctgctgctgtcccttctccagtttttgaataactgatggtcgaactgaaacctcctgcgtgccttcctgagatttatgaggtctggaatgtaactcttcaataggttctgaaacctcggatggtctctcttcggtagcatcctcatcctcaaccttatcctcatcctcttcctcttcttcagaaaaagcatcatccaaatgcaccacttcagacgatgacccagtattcacatgtgtctcatcttgtgttgaactgctctcttgacaatgatatgggtggtgctgcagtacatcctgtaagaaacgttccatcaaactactggtacatatttgacgtctactctgtctggtcaaactcctgtgctgagcactgaacaaatgctgttccaggttattatactgcacacggcaataactgcaatatccttgtcttttctgcatcttgaataaataactgaagtcagatggctactgtctttgaatactcaagttaaaatttggtctcttttccactaatttacttcacttattaacctggagcagaaaaggtcaggtatttcatcagctgtattagttctggcaagtatctgcgaggcggccgcgggagcccagcgagcggtcctggcgtccctcgggaagaaggcgccccgggcgcccggcgagcag

SEQ ID NO: 18372 - RNA, 9654 nt, Homo sapiens
  source 1..9654: mol_type = other RNA
tgaagtaccagctactcgagaggcttaggcaggagaattgcttgaacccgggaggtggaggttgcggtgagctaagttcaggccactgcactccagcctgggcaagacagtgagactctgtctcaaaaaataataataataaataaacataaaaataaaaactgatatggtaatgcctaaaatatttttaggggataaggccacaaaataacctggattttcatattaagccaccaactcttcatgtagaagagagtaaaggtggttaaaaaaaagggggggaatgcctaaacacatgggcaaaattattttcccctttaagatctaataaggctaacccaaaaaacctagagactgtatgtgtgcatgtgtccaaatgataaaagttagagacttgcagatccaatttaaatgaagcaggaggagtttgtgctatgcataaaaaaaatcaccagtttttaaaaactgtattaaagattatggaatctcattttctggaatgctttaaaaagaaagaaaacttatattttgtttgtattcatttaagtcaaccccattcaaaagttgacataattcattataattccttctttttaataagtttgctatattcattctcacaatgttaaatttgctggcatgagagagataatcataaaaaataagagggatatgatttgaggaacaaaattctatatacggtgctaaattattttgtgacataaattaagatgaagttcttctacagaaaatgttggacaaaggctgtttctgaatcttaaaatgaaaggactctaaacactaattttaaatgaatataaaaattctgaaaaataatatttatagcaaaatagttcaagattagttttctcaccaaagctgggaaagctgtgtgcacaaagtaccaaatatatttcaactgaagtactgaatcctcaactagcctgaacacaaaaccaacttctattttacctcattacctctcagtttgtttgctagccgagtcatcattctctcacgttgttgtaaacaagatgagcttctcagatcatatgctctcacaggtgtagaaggacctttctgtcggccatggtagctttcatcagtcttcttcctccttcttgcaacgcggcaagaagcccgcacaggtcgctttggaggaggatttgccatagcgcttgacagctcttcggcaccagctggtggaactgaagagttcaaaagcactttagctgttctcttcgccttctttagcctactgacaacagattttttcttcttcagataccttccaagaaaagcgctcctggactgatatctatgacgtaaaaagacagagtatttcgaaatatactttctaatgatatcacttggtttggtccgaatccaaattgactgtttctctgaagcttttctgggtttttgctggagaataattggtttataaacctttttgggaaaacctagcttattactactagttgtcaccctctttccatgaattttctttttactttgactttccaaaagcttatttctaactgattttggagagattttgacaacatcatgatttaaaaatgttagctggaaatttcttttctttggaagctcacgagcatgcagaacctttgattcttccagaaacagagaagagtcactggttccctgatgtgaattaaatccatatcttgccggcactgccattaaaggcgctgaagcagagccttgtccatcagcatcattatctcctgcactggagttttggttgctcctattaaaatgaattttaacccagttacgcctctcaaactctggtactattacactcaggggaggactaattacaatttgcttaatcaagggctcataataatcaaagatattccgtttatatttgcatataaaccgaatatcattatcccaactatggtgcctcattttagggaaaggaaggccttcaccctctttcagtttaatatttaaagaagaaagaacacagactaaggctttgggttgcataggcttcaaaactttagtacatgatgcaggaaattcaactgtcccaattttgactttctttttggtttttctgtcatcctgtaaacgtgaacacttactttttggtgggtcttcctcttgtctaattatttttcttttcatcactgggtaattcttacaactggtctgagtactatggctgattttcgctgtctggcattgagaagccacacgccccttttgcttaggaggcctctctgctggaggatgacgatggcatggtttatctaaggccactgacaagtcatcaatatctgaaataccacagacaatatcatcactctctgacacagcttgagttggtgcagtgtcctccttaccttgcaagtcagcccaggtaaccttttttttccccttcgaagaaacttttttggtctcacagtcatcatcaaagtaacagtggaaacgaccttccctaaactccttcaccagagcattaatttttatgtcatcttctctcattatctgagaccatgttttccccacaaatgaaggaggtacatgaggcaaggcttcaagaactggttcatcaggattatcctctatgacatcctttgcttttttcaggttccttacagaatcaaccttgagaacagagcttgactgggaatcatggttcttttctttcaagtcagaagataccttcttacaagggtgtcttttcttaacagtttcttgaggctgatcagtatcagatggaagagggggagcacactgaaaattcatctcaaaaccatccggttcacagctcacttctagatctctatgttttagcttcgaacgtttttttttatcagcccttcgatggagcgctgacttggaagaggcaccaaaatccactgcagaagcactagactgacagctcttaccttttaggccagcatttcttggatccttccgaagactggcttctttgtgagctttctgcagtcggtgagtcgttcgatgagaagtgtcttccaaattaaattttcctttagaaccattatatccacagctcttatcttctgaatcaatatatttcaccattttctcatcaggtccttgtgactcgtaagtcatggactgatcagaggcatcaacattaaaattcatttcagaaccacaagattgacaacttggctctcccagaataatatagtccttcttccggtttattattttgaaagtctctttgcattggtttgtcattgagggagtagaggctttacaattacatctgacttcagaaccaaaaaagtcacagctcttatcttctatatcaatacattctgtatttatacagctgatatctttgacagtcaactgaggtgggtcagtcactaactgaaggggaatatcatctgaaattacttcataatcactatcaccgggcaccagatccacaagtaccacctttggaaggtgggtttctttgactgatcctggaaattggttaactactatttgaaaaggaacatcagaatcatacatcatttctgaatcactaggttgatcggtcttttcttccatgacaacatgctcttccttctgaaggtctgcctctttgtaagacacttgaggttggtcaacttctgactgaagatgaacacaagaatgacattttatttcagaaccacagacttcacagttcttattttctagatcattatgatccttcttttgcaagtttatttctttgacaggtacagaagattgatcagtcacaaactgaacaggaatatgagaagcataacttacatcaaaatcacctaatttatagctcttatcttccaggtaaatatggtcttccttccaaagatttatttctttgacaggtttttgaagctcatctgctgctgcctgaaaagagtcattggaatcagaactttcttcaggactataagaattactgctcttatcttccagactggcatgctcctcttccaaaatgtgtggttgttttatcactgactgaagagggatatttgaaacataaattatttcagaatcactgggcacatagcccttatcatccagacaaacatgttcctccctcaaaagatttatttctttattcgcccctggaattttattagttacggactgaaggggttcatgagaatcaaaatttattctggaatctgtaggtttgacaatcttattttccaagtcaacatgctctttccaaagactgacctccttaactacttcttcaggttggccagccactggctgaagaacatcagaatcatacataatttcaaaacccttagcttcatttctcctatcttccgtgtcaacttcttcatccttccaaaggcttatttctttaacggtttctctcagccggtcagccactgactgaagagggtcatcagaatcaaaacttacttcagaaccacaacattgattgtgcttaccttctagttcaatgtgctcctgctccaaaatagttatttgaggtcgattgactattgactgacccaagaaaccagaatccaaattcatttctgaacaactatattggctgttcttaacttccaagtacatatggttttcattcccaaggttcacatgtttaatagctactttgggttgatcagccacagattggacagaaacatcaggatgatgtattaatttataagtactaggttcattaatcttatttttcaggccaataacctcttccttccattggtctatttttttaaccgcttcctgaagttgttcagaatcaaaagttattttagaatcacctgatttactgtttttgtccttcagattaacatgtttttccttcaaaaaagctagttgaggttggtcagtcattgactgaggtggaacattagaatccaaaattatttcagaaccactacatttatcattcttgttttctagaacatattgcttctttctgtttattttgttaacagctacttgaggttcagttactgaataatgagggacaccagaatctaaacttgtttttgaaccactgaattcagtacttctaccttggaattcagcgtgcttttctctttgaagccatgtttctttgacaattacttcaggtttgtgagtcgctgcctgaagagggacatcagaatccaaacttgtttcaaaaacactcttattttctaagtacatgtgctcttttgtgtgaaggcttatttctttaatgggatcttcagaacgtccagtcactgaatgaaaaatgatattataatccaaacttacttcagaatcaataggttcattttccttattttctaagtgtacctgctcttctttttgaggatttagctttttaacagctacttcgggagaattagtcactgaatgaagaggggcatgggaatccgaacttatttcagaaccactgggttcatcattcttcctttctaagtgaatgtactcttctttctgaattacttctttaacagctacttcagggtgatcatttcctgaatgaagaggaatatcagaatcaaaagttatttcagagacacaagattcattacttttactttccagatcaacagtttcttcctcataaacagctacttcaggttggtcaattactgaataaagaggaatatcagaatcaaaagttatttcagaactatctgactcacagctctcatcttccaggtcaatgtgccgttcttttccttcagcatccagatgagactgctcagtaactgacagaagaggcgggtcagaatcaaaagtcaactcagagctggagcaatcatagctcctaacttccatgtcaatatttaactctttaagatttacttcatccaaagcttcttgaggctcatcatgagctgaatgataaagagaagccggagaatcagaactcagagaagaacggctagactgaacactcttattctcaaggtcaacatccactttctgacgctctatttcggctacttgagactggtcagctaattgagcatcagcctgaaaacccatttcaggaccatgggattcacagttcatatccataaggtcagcattcttctccttcagaagatttatcttttcaacagccctctgggattcatctgcaactgtcccaagtgagacatcacaatcaagatgtgctttagcactactgggtttacgcttcttatgttttaggtggacttgtctacctttcaggtttcttcctttgacagtcagttggggatgatcaactactgactcaagagaaacatcacaatcaaaacttgtttcagaacaactcgatccatagttatcaaccaagctggtatgagccttcttccgaagttttgtttctgtgacagccactgggggtctgtcaaccactgactgcagtgggaaaacagaatcagcacttacttcagagctactggaaccatagttcttatcaaccaaaccaatgtgcacttccttaggaaggtttacttctgttacagattgttgggggtagtcactagtggactgaggtgaagcatcacaatcaaaattcgtttcagaactactagattcatagctttggtcaaccaggctaatatgccttgcattctgaagacttatttctttaacaatcatttgggattggttggtaaccaagtgaagaatgtcatcacaatcagaacttattttagaaacataagatttattattcttatactgtacatcagtacgtacttccttggaaaggtttacttctttggcactcactttagattggtcagtcagtgaatgaaaagaggaactgcaatcaaaactcatttctgaacctctagactcatagttatcttcttggtcaatttgctcctccttccaaagacttaagtcttgtgcagtctcttggggctgatcagatgctgactgaagagagatacaatcaaacttcatttcagaactcactgagcacttctgttcccaaaaggctgtcttgttaaaaaccaaatgcttttcttcttgggtacaatccatgttagaaaagaattcctcatggttctttgcaatagtatcttcaaagattcctttattagaaggcatgtcagttttattcgggtttactgctaatttggaaggagatttaactcttaaggagcccttagtacccatgcgttcatggaatttcaagccagctgataaagttttaccctgagattttacatctttccacaaaaccaacttatctgaattcatgcgtaaagatttcctatttgattctttatgtttctgatacgaaaatgaagtagtttctacatgggatgatggcacaggatttctagaggccccatctggctgttcaagatatttctcaactttgtttgggtcacatttgctaactgaatccaaatgagctgctggtggtaaactagttgtattagctgtaactggtctatcgttagagctttcaggtaaacaactagcaggagcattacaaatcactggggggcgtaccaagttgcttctattatttgtagcctgaccaatatctactaggttacattttctcacactggccccaattttatgaacaaactccaagggctgctgctgtcccttctccagtttttgaataactgatggtcgaactgaaacctcctgcgtgccttcctgagatttatgaggtctggaatgtaactcttcaataggttctgaaacctcggatggtctctcttcggtagcatcctcatcctcaaccttatcctcatcctcttcctcttcttcagaaaaagcatcatccaaatgcaccacttcagacgatgacccagtattcacatgtgtctcatcttgtgttgaactgctctcttgacaatgatatgggtggtgctgcagtacatcctgtaagaaacgttccatcaaactactggtacatatttgacgtctactctgtctggtcaaactcctgtgctgagcactgaacaaatgctttccactgttcttcattacttcctgtatctctgagcttccatcgggaatcattttccttctgcctgaagaactcctttttagtttttcctttagtgagagtctgctgttccaggttattatactgcacacggcaataactgcaatatccttgtcttttctgcatcttgaataaataactgaagtcagatggctactgtctttgaatactcaagttaaaatttggtctcttttccactaatttacttcacttattaacctggagcagaaaaggtcaggtatttcatcagctgtattagttctggcaagtatctccgcggaggctgcccggattccttccgggccgcggtggagaccgaggaccgagccgggcgctctcccttcttattccggttccgcggcggcgcccgaatcccagaccgtccgagcgccacggccccgctgcccgcggagccagaaataggcgacttcggcccctgcggtccggaggcgagaagcggcgcgggagcgcgtctctcaggacgcgggccccgagtcgcgactccactcacgcaggcatccaaggcaacgtggcgttgcaaccctgatggaggtttgacgtcagggaaggtgcgaaaaccagaccccttctgacgcaggagcggcgggaccgccccctgcccgcccacccactcactcactctcccacccgggcggaggagccccttcctcccctccagaagctcttaaagcggacacttcctccctggtcagggccccactccggagcttgggaaatctatcgcgttccaacaaaaatgactagactcataagcacagttgggacgcgaagtagagaccaaggttttagcgtttgagggtccaaataaaaactgcttgccaattcaaagcaacgtatgaatgtagaaaagaaaacggggctaagagagctagtcgtttccgtttccatgcctatttcatagtgaggtgcatctcacaaaagctgctgttcaatgagcgcttgctctgtgctaggcaccgtttaaggtttctatacattattgcatttcatttcagagtaactctgaatgaatcctattattgtccccctttgacaaattgagaaaactgaggcttaaggaagttaggtattcaaagatctatcctgcacattaaagggttacaaatattaacaaacaacattaggtcatgcaattatattcactgcgctaccccattacgaatatagttgtgagcaaaaacagtttaagtgtaacggagatcacaaacctaaatgaatcacactactgaatatgaaattataatctgcgataagaaggttctgaaacacctaaaccaattttactaaaatggagagaggccctgttgcaaagcttatgtctaatgtaaaaataatcttaaaatgagctactttgctctttggctgtagctgtaattgtcgttaccctttttagtaagcttgtgattttgtccctttaaagaacaacaacaaaaaaacttgcctattgcttttgcgtccattgtttttattctttctgtatttctcagctccttcttcccccactacatctttctctcactttaaagttgggctcctgcaactgttcgatttataacctcccttagatttaacataccaaaaagtacggatttcttttaaggcaagttttttccacatcccaactt

SEQ ID NO: 18373 - RNA, 8468 nt, Homo sapiens
  source 1..8468: mol_type = other RNA
tgaagtaccagctactcgagaggcttaggcaggagaattgcttgaacccgggaggtggaggttgcggtgagctaagttcaggccactgcactccagcctgggcaagacagtgagactctgtctcaaaaaataataataataaataaacataaaaataaaaactgatatggtaatgcctaaaatatttttaggggataaggccacaaaataacctggattttcatattaagccaccaactcttcatgtagaagagagtaaaggtggttaaaaaaaagggggggaatgcctaaacacatgggcaaaattattttcccctttaagatctaataaggctaacccaaaaaacctagagactgtatgtgtgcatgtgtccaaatgataaaagttagagacttgcagatccaatttaaatgaagcaggaggagtttgtgctatgcataaaaaaaatcaccagtttttaaaaactgtattaaagattatggaatctcattttctggaatgctttaaaaagaaagaaaacttatattttgtttgtattcatttaagtcaaccccattcaaaagttgacataattcattataattccttctttttaataagtttgctatattcattctcacaatgttaaatttgctggcatgagagagataatcataaaaaataagagggatatgatttgaggaacaaaattctatatacggtgctaaattattttgtgacataaattaagatgaagttcttctacagaaaatgttggacaaaggctgtttctgaatcttaaaatgaaaggactctaaacactaattttaaatgaatataaaaattctgaaaaataatatttatagcaaaatagttcaagattagttttctcaccaaagctgggaaagctgtgtgcacaaagtaccaaatatatttcaactgaagtactgaatcctcaactagcctgaacacaaaaccaacttctattttacctcattacctctcagtttgtttgctagccgagtcatcattctctcacgttgttgtaaacaagatgagcttctcagatcatatgctctcacaggtgtagaaggacctttctgtcggccatggtagctttcatcagtcttcttcctccttcttgcaacgcggcaagaagcccgcacaggtcgctttggaggaggatttgccatagcgcttgacagctcttcggcaccagctggtggaactgaagagttcaaaagcactttagctgttctcttcgccttctttagcctactgacaacagattttttcttcttcagataccttccaagaaaagcgctcctggactgatatctatgacgtaaaaagacagagtatttcgaaatatactttctaatgatatcacttggtttggtccgaatccaaattgactgtttctctgaagcttttctgggtttttgctggagaataattggtttataaacctttttgggaaaacctagcttattactactagttgtcaccctctttccatgaattttctttttactttgactttccaaaagcttatttctaactgattttggagagattttgacaacatcatgatttaaaaatgttagctggaaatttcttttctttggaagctcacgagcatgcagaacctttgattcttccagaaacagagaagagtcactggttccctgatgtgaattaaatccatatcttgccggcactgccattaaaggcgctgaagcagagccttgtccatcagcatcattatctcctgcactggagttttggttgctcctattaaaatgaattttaacccagttacgcctctcaaactctggtactattacactcaggggaggactaattacaatttgcttaatcaagggctcataataatcaaagatattccgtttatatttgcatataaaccgaatatcattatcccaactatggtgcctcattttagggaaaggaaggccttcaccctctttcagtttaatatttaaagaagaaagaacacagactaaggctttgggttgcataggcttcaaaactttagtacatgatgcaggaaattcaactgtcccaattttgactttctttttggtttttctgtcatcctgtaaacgtgaacacttactttttggtgggtcttcctcttgtctaattatttttcttttcatcactgggtaattcttacaactggtctgagtactatggctgattttcgctgtctggcattgagaagccacacgccccttttgcttaggaggcctctctgctggaggatgacgatggcatggtttatctaaggccactgacaagtcatcaatatctgaaataccacagacaatatcatcactctctgacacagcttgagttggtgcagtgtcctccttaccttgcaagtcagcccaggtaaccttttttttccccttcgaagaaacttttttggtctcacagtcatcatcaaagtaacagtggaaacgaccttccctaaactccttcaccagagcattaatttttatgtcatcttctctcattatctgagaccatgttttccccacaaatgaaggaggtacatgaggcaaggcttcaagaactggttcatcaggattatcctctatgacatcctttgcttttttcaggttccttacagaatcaaccttgagaacagagcttgactgggaatcatggttcttttctttcaagtcagaagataccttcttacaagggtgtcttttcttaacagtttcttgaggctgatcagtatcagatggaagagggggagcacactgaaaattcatctcaaaaccatccggttcacagctcacttctagatctctatgttttagcttcgaacgtttttttttatcagcccttcgatggagcgctgacttggaagaggcaccaaaatccactgcagaagcactagactgacagctcttaccttttaggccagcatttcttggatccttccgaagactggcttctttgtgagctttctgcagtcggtgagtcgttcgatgagaagtgtcttccaaattaaattttcctttagaaccattatatccacagctcttatcttctgaatcaatatatttcaccattttctcatcaggtccttgtgactcgtaagtcatggactgatcagaggcatcaacattaaaattcatttcagaaccacaagattgacaacttggctctcccagaataatatagtccttcttccggtttattattttgaaagtctctttgcattggtttgtcattgagggagtagaggctttacaattacatctgacttcagaaccaaaaaagtcacagctcttatcttctatatcaatacattctgtatttatacagctgatatctttgacagtcaactgaggtgggtcagtcactaactgaaggggaatatcatctgaaattacttcataatcactatcaccgggcaccagatccacaagtaccacctttggaaggtgggtttctttgactgatcctggaaattggttaactactatttgaaaaggaacatcagaatcatacatcatttctgaatcactaggttgatcggtcttttcttccatgacaacatgctcttccttctgaaggtctgcctctttgtaagacacttgaggttggtcaacttctgactgaagatgaacacaagaatgacattttatttcagaaccacagacttcacagttcttattttctagatcattatgatccttcttttgcaagtttatttctttgacaggtacagaagattgatcagtcacaaactgaacaggaatatgagaagcataacttacatcaaaatcacctaatttatagctcttatcttccaggtaaatatggtcttccttccaaagatttatttctttgacaggtttttgaagctcatctgctgctgcctgaaaagagtcattggaatcagaactttcttcaggactataagaattactgctcttatcttccagactggcatgctcctcttccaaaatgtgtggttgttttatcactgactgaagagggatatttgaaacataaattatttcagaatcactgggcacatagcccttatcatccagacaaacatgttcctccctcaaaagatttatttctttattcgcccctggaattttattagttacggactgaaggggttcatgagaatcaaaatttattctggaatctgtaggtttgacaatcttattttccaagtcaacatgctctttccaaagactgacctccttaactacttcttcaggttggccagccactggctgaagaacatcagaatcatacataatttcaaaacccttagcttcatttctcctatcttccgtgtcaacttcttcatccttccaaaggcttatttctttaacggtttctctcagccggtcagccactgactgaagagggtcatcagaatcaaaacttacttcagaaccacaacattgattgtgcttaccttctagttcaatgtgctcctgctccaaaatagttatttgaggtcgattgactattgactgacccaagaaaccagaatccaaattcatttctgaacaactatattggctgttcttaacttccaagtacatatggttttcattcccaaggttcacatgtttaatagctactttgggttgatcagccacagattggacagaaacatcaggatgatgtattaatttataagtactaggttcattaatcttatttttcaggccaataacctcttccttccattggtctatttttttaaccgcttcctgaagttgttcagaatcaaaagttattttagaatcacctgatttactgtttttgtccttcagattaacatgtttttccttcaaaaaagctagttgaggttggtcagtcattgactgaggtggaacattagaatccaaaattatttcagaaccactacatttatcattcttgttttctagaacatattgcttctttctgtttattttgttaacagctacttgaggttcagttactgaataatgagggacaccagaatctaaacttgtttttgaaccactgaattcagtacttctaccttggaattcagcgtgcttttctctttgaagccatgtttctttgacaattacttcaggtttgtgagtcgctgcctgaagagggacatcagaatccaaacttgtttcaaaaacactcttattttctaagtacatgtgctcttttgtgtgaaggcttatttctttaatgggatcttcagaacgtccagtcactgaatgaaaaatgatattataatccaaacttacttcagaatcaataggttcattttccttattttctaagtgtacctgctcttctttttgaggatttagctttttaacagctacttcgggagaattagtcactgaatgaagaggggcatgggaatccgaacttatttcagaaccactgggttcatcattcttcctttctaagtgaatgtactcttctttctgaattacttctttaacagctacttcagggtgatcatttcctgaatgaagaggaatatcagaatcaaaagttatttcagagacacaagattcattacttttactttccagatcaacagtttcttcctcataaacagctacttcaggttggtcaattactgaataaagaggaatatcagaatcaaaagttatttcagaactatctgactcacagctctcatcttccaggtcaatgtgccgttcttttccttcagcatccagatgagactgctcagtaactgacagaagaggcgggtcagaatcaaaagtcaactcagagctggagcaatcatagctcctaacttccatgtcaatatttaactctttaagatttacttcatccaaagcttcttgaggctcatcatgagctgaatgataaagagaagccggagaatcagaactcagagaagaacggctagactgaacactcttattctcaaggtcaacatccactttctgacgctctatttcggctacttgagactggtcagctaattgagcatcagcctgaaaacccatttcaggaccatgggattcacagttcatatccataaggtcagcattcttctccttcagaagatttatcttttcaacagccctctgggattcatctgcaactgtcccaagtgagacatcacaatcaagatgtgctttagcactactgggtttacgcttcttatgttttaggtggacttgtctacctttcaggtttcttcctttgacagtcagttggggatgatcaactactgactcaagagaaacatcacaatcaaaacttgtttcagaacaactcgatccatagttatcaaccaagctggtatgagccttcttccgaagttttgtttctgtgacagccactgggggtctgtcaaccactgactgcagtgggaaaacagaatcagcacttacttcagagctactggaaccatagttcttatcaaccaaaccaatgtgcacttccttaggaaggtttacttctgttacagattgttgggggtagtcactagtggactgaggtgaagcatcacaatcaaaattcgtttcagaactactagattcatagctttggtcaaccaggctaatatgccttgcattctgaagacttatttctttaacaatcatttgggattggttggtaaccaagtgaagaatgtcatcacaatcagaacttattttagaaacataagatttattattcttatactgtacatcagtacgtacttccttggaaaggtttacttctttggcactcactttagattggtcagtcagtgaatgaaaagaggaactgcaatcaaaactcatttctgaacctctagactcatagttatcttcttggtcaatttgctcctccttccaaagacttaagtcttgtgcagtctcttggggctgatcagatgctgactgaagagagatacaatcaaacttcatttcagaactcactgagcacttctgttcccaaaaggctgtcttgttaaaaaccaaatgcttttcttcttgggtacaatccatgttagaaaagaattcctcatggttctttgcaatagtatcttcaaagattcctttattagaaggcatgtcagttttattcgggtttactgctaatttggaaggagatttaactcttaaggagcccttagtacccatgcgttcatggaatttcaagccagctgataaagttttaccctgagattttacatctttccacaaaaccaacttatctgaattcatgcgtaaagatttcctatttgattctttatgtttctgatacgaaaatgaagtagtttctacatgggatgatggcacaggatttctagaggccccatctggctgttcaagatatttctcaactttgtttgggtcacatttgctaactgaatccaaatgagctgctggtggtaaactagttgtattagctgtaactggtctatcgttagagctttcaggtaaacaactagcaggagcattacaaatcactggggggcgtaccaagttgcttctattatttgtagcctgaccaatatctactaggttacattttctcacactggccccaattttatgaacaaactccaagggctgctgctgtcccttctccagtttttgaataactgatggtcgaactgaaacctcctgcgtgccttcctgagatttatgaggtctggaatgtaactcttcaataggttctgaaacctcggatggtctctcttcggtagcatcctcatcctcaaccttatcctcatcctcttcctcttcttcagaaaaagcatcatccaaatgcaccacttcagacgatgacccagtattcacatgtgtctcatcttgtgttgaactgctctcttgacaatgatatgggtggtgctgcagtacatcctgtaagaaacgttccatcaaactactggtacatatttgacgtctactctgtctggtcaaactcctgtgctgagcactgaacaaatgctttccactgttcttcattacttcctgtatctctgagcttccatcgggaatcattttccttctgcctgaagaactcctttttagtttttcctttagtgagagtctgctgttccaggttattatactgcacacggcaataactgcaatatccttgtcttttctgcatcttgaataaataactgaagtcagatggctactgtctttgaatactcaagttaaaatttggtctcttttccactaatttacttcacttattaacctggagcagaaaaggtcaggtatttcatcagctgtattagttctggcaagtatctccttccctcgccccgccacctcgatcccggcccggagccgccgacacctctcacgcagcaggggcagaaagggacgcggggtggggggaagccgaggacctgcgaggcggccgcgggagcccagcgagcggtcctggcgtccctcgggaagaaggcgccccgggcgcccggcgagcaggccccgcc

SEQ ID NO: 18374 - RNA, 8347 nt, Homo sapiens
  source 1..8347: mol_type = other RNA
tgaagtaccagctactcgagaggcttaggcaggagaattgcttgaacccgggaggtggaggttgcggtgagctaagttcaggccactgcactccagcctgggcaagacagtgagactctgtctcaaaaaataataataataaataaacataaaaataaaaactgatatggtaatgcctaaaatatttttaggggataaggccacaaaataacctggattttcatattaagccaccaactcttcatgtagaagagagtaaaggtggttaaaaaaaagggggggaatgcctaaacacatgggcaaaattattttcccctttaagatctaataaggctaacccaaaaaacctagagactgtatgtgtgcatgtgtccaaatgataaaagttagagacttgcagatccaatttaaatgaagcaggaggagtttgtgctatgcataaaaaaaatcaccagtttttaaaaactgtattaaagattatggaatctcattttctggaatgctttaaaaagaaagaaaacttatattttgtttgtattcatttaagtcaaccccattcaaaagttgacataattcattataattccttctttttaataagtttgctatattcattctcacaatgttaaatttgctggcatgagagagataatcataaaaaataagagggatatgatttgaggaacaaaattctatatacggtgctaaattattttgtgacataaattaagatgaagttcttctacagaaaatgttggacaaaggctgtttctgaatcttaaaatgaaaggactctaaacactaattttaaatgaatataaaaattctgaaaaataatatttatagcaaaatagttcaagattagttttctcaccaaagctgggaaagctgtgtgcacaaagtaccaaatatatttcaactgaagtactgaatcctcaactagcctgaacacaaaaccaacttctattttacctcattacctctcagtttgtttgctagccgagtcatcattctctcacgttgttgtaaacaagatgagcttctcagatcatatgctctcacaggtgtagaaggacctttctgtcggccatggtagctttcatcagtcttcttcctccttcttgcaacgcggcaagaagcccgcacaggtcgctttggaggaggatttgccatagcgcttgacagctcttcggcaccagctggtggaactgaagagttcaaaagcactttagctgttctcttcgccttctttagcctactgacaacagattttttcttcttcagataccttccaagaaaagcgctcctggactgatatctatgacgtaaaaagacagagtatttcgaaatatactttctaatgatatcacttggtttggtccgaatccaaattgactgtttctctgaagcttttctgggtttttgctggagaataattggtttataaacctttttgggaaaacctagcttattactactagttgtcaccctctttccatgaattttctttttactttgactttccaaaagcttatttctaactgattttggagagattttgacaacatcatgatttaaaaatgttagctggaaatttcttttctttggaagctcacgagcatgcagaacctttgattcttccagaaacagagaagagtcactggttccctgatgtgaattaaatccatatcttgccggcactgccattaaaggcgctgaagcagagccttgtccatcagcatcattatctcctgcactggagttttggttgctcctattaaaatgaattttaacccagttacgcctctcaaactctggtactattacactcaggggaggactaattacaatttgcttaatcaagggctcataataatcaaagatattccgtttatatttgcatataaaccgaatatcattatcccaactatggtgcctcattttagggaaaggaaggccttcaccctctttcagtttaatatttaaagaagaaagaacacagactaaggctttgggttgcataggcttcaaaactttagtacatgatgcaggaaattcaactgtcccaattttgactttctttttggtttttctgtcatcctgtaaacgtgaacacttactttttggtgggtcttcctcttgtctaattatttttcttttcatcactgggtaattcttacaactggtctgagtactatggctgattttcgctgtctggcattgagaagccacacgccccttttgcttaggaggcctctctgctggaggatgacgatggcatggtttatctaaggccactgacaagtcatcaatatctgaaataccacagacaatatcatcactctctgacacagcttgagttggtgcagtgtcctccttaccttgcaagtcagcccaggtaaccttttttttccccttcgaagaaacttttttggtctcacagtcatcatcaaagtaacagtggaaacgaccttccctaaactccttcaccagagcattaatttttatgtcatcttctctcattatctgagaccatgttttccccacaaatgaaggaggtacatgaggcaaggcttcaagaactggttcatcaggattatcctctatgacatcctttgcttttttcaggttccttacagaatcaaccttgagaacagagcttgactgggaatcatggttcttttctttcaagtcagaagataccttcttacaagggtgtcttttcttaacagtttcttgaggctgatcagtatcagatggaagagggggagcacactgaaaattcatctcaaaaccatccggttcacagctcacttctagatctctatgttttagcttcgaacgtttttttttatcagcccttcgatggagcgctgacttggaagaggcaccaaaatccactgcagaagcactagactgacagctcttaccttttaggccagcatttcttggatccttccgaagactggcttctttgtgagctttctgcagtcggtgagtcgttcgatgagaagtgtcttccaaattaaattttcctttagaaccattatatccacagctcttatcttctgaatcaatatatttcaccattttctcatcaggtccttgtgactcgtaagtcatggactgatcagaggcatcaacattaaaattcatttcagaaccacaagattgacaacttggctctcccagaataatatagtccttcttccggtttattattttgaaagtctctttgcattggtttgtcattgagggagtagaggctttacaattacatctgacttcagaaccaaaaaagtcacagctcttatcttctatatcaatacattctgtatttatacagctgatatctttgacagtcaactgaggtgggtcagtcactaactgaaggggaatatcatctgaaattacttcataatcactatcaccgggcaccagatccacaagtaccacctttggaaggtgggtttctttgactgatcctggaaattggttaactactatttgaaaaggaacatcagaatcatacatcatttctgaatcactaggttgatcggtcttttcttccatgacaacatgctcttccttctgaaggtctgcctctttgtaagacacttgaggttggtcaacttctgactgaagatgaacacaagaatgacattttatttcagaaccacagacttcacagttcttattttctagatcattatgatccttcttttgcaagtttatttctttgacaggtacagaagattgatcagtcacaaactgaacaggaatatgagaagcataacttacatcaaaatcacctaatttatagctcttatcttccaggtaaatatggtcttccttccaaagatttatttctttgacaggtttttgaagctcatctgctgctgcctgaaaagagtcattggaatcagaactttcttcaggactataagaattactgctcttatcttccagactggcatgctcctcttccaaaatgtgtggttgttttatcactgactgaagagggatatttgaaacataaattatttcagaatcactgggcacatagcccttatcatccagacaaacatgttcctccctcaaaagatttatttctttattcgcccctggaattttattagttacggactgaaggggttcatgagaatcaaaatttattctggaatctgtaggtttgacaatcttattttccaagtcaacatgctctttccaaagactgacctccttaactacttcttcaggttggccagccactggctgaagaacatcagaatcatacataatttcaaaacccttagcttcatttctcctatcttccgtgtcaacttcttcatccttccaaaggcttatttctttaacggtttctctcagccggtcagccactgactgaagagggtcatcagaatcaaaacttacttcagaaccacaacattgattgtgcttaccttctagttcaatgtgctcctgctccaaaatagttatttgaggtcgattgactattgactgacccaagaaaccagaatccaaattcatttctgaacaactatattggctgttcttaacttccaagtacatatggttttcattcccaaggttcacatgtttaatagctactttgggttgatcagccacagattggacagaaacatcaggatgatgtattaatttataagtactaggttcattaatcttatttttcaggccaataacctcttccttccattggtctatttttttaaccgcttcctgaagttgttcagaatcaaaagttattttagaatcacctgatttactgtttttgtccttcagattaacatgtttttccttcaaaaaagctagttgaggttggtcagtcattgactgaggtggaacattagaatccaaaattatttcagaaccactacatttatcattcttgttttctagaacatattgcttctttctgtttattttgttaacagctacttgaggttcagttactgaataatgagggacaccagaatctaaacttgtttttgaaccactgaattcagtacttctaccttggaattcagcgtgcttttctctttgaagccatgtttctttgacaattacttcaggtttgtgagtcgctgcctgaagagggacatcagaatccaaacttgtttcaaaaacactcttattttctaagtacatgtgctcttttgtgtgaaggcttatttctttaatgggatcttcagaacgtccagtcactgaatgaaaaatgatattataatccaaacttacttcagaatcaataggttcattttccttattttctaagtgtacctgctcttctttttgaggatttagctttttaacagctacttcgggagaattagtcactgaatgaagaggggcatgggaatccgaacttatttcagaaccactgggttcatcattcttcctttctaagtgaatgtactcttctttctgaattacttctttaacagctacttcagggtgatcatttcctgaatgaagaggaatatcagaatcaaaagttatttcagagacacaagattcattacttttactttccagatcaacagtttcttcctcataaacagctacttcaggttggtcaattactgaataaagaggaatatcagaatcaaaagttatttcagaactatctgactcacagctctcatcttccaggtcaatgtgccgttcttttccttcagcatccagatgagactgctcagtaactgacagaagaggcgggtcagaatcaaaagtcaactcagagctggagcaatcatagctcctaacttccatgtcaatatttaactctttaagatttacttcatccaaagcttcttgaggctcatcatgagctgaatgataaagagaagccggagaatcagaactcagagaagaacggctagactgaacactcttattctcaaggtcaacatccactttctgacgctctatttcggctacttgagactggtcagctaattgagcatcagcctgaaaacccatttcaggaccatgggattcacagttcatatccataaggtcagcattcttctccttcagaagatttatcttttcaacagccctctgggattcatctgcaactgtcccaagtgagacatcacaatcaagatgtgctttagcactactgggtttacgcttcttatgttttaggtggacttgtctacctttcaggtttcttcctttgacagtcagttggggatgatcaactactgactcaagagaaacatcacaatcaaaacttgtttcagaacaactcgatccatagttatcaaccaagctggtatgagccttcttccgaagttttgtttctgtgacagccactgggggtctgtcaaccactgactgcagtgggaaaacagaatcagcacttacttcagagctactggaaccatagttcttatcaaccaaaccaatgtgcacttccttaggaaggtttacttctgttacagattgttgggggtagtcactagtggactgaggtgaagcatcacaatcaaaattcgtttcagaactactagattcatagctttggtcaaccaggctaatatgccttgcattctgaagacttatttctttaacaatcatttgggattggttggtaaccaagtgaagaatgtcatcacaatcagaacttattttagaaacataagatttattattcttatactgtacatcagtacgtacttccttggaaaggtttacttctttggcactcactttagattggtcagtcagtgaatgaaaagaggaactgcaatcaaaactcatttctgaacctctagactcatagttatcttcttggtcaatttgctcctccttccaaagacttaagtcttgtgcagtctcttggggctgatcagatgctgactgaagagagatacaatcaaacttcatttcagaactcactgagcacttctgttcccaaaaggctgtcttgttaaaaaccaaatgcttttcttcttgggtacaatccatgttagaaaagaattcctcatggttctttgcaatagtatcttcaaagattcctttattagaaggcatgtcagttttattcgggtttactgctaatttggaaggagatttaactcttaaggagcccttagtacccatgcgttcatggaatttcaagccagctgataaagttttaccctgagattttacatctttccacaaaaccaacttatctgaattcatgcgtaaagatttcctatttgattctttatgtttctgatacgaaaatgaagtagtttctacatgggatgatggcacaggatttctagaggccccatctggctgttcaagatatttctcaactttgtttgggtcacatttgctaactgaatccaaatgagctgctggtggtaaactagttgtattagctgtaactggtctatcgttagagctttcaggtaaacaactagcaggagcattacaaatcactggggggcgtaccaagttgcttctattatttgtagcctgaccaatatctactaggttacattttctcacactggccccaattttatgaacaaactccaagggctgctgctgtcccttctccagtttttgaataactgatggtcgaactgaaacctcctgcgtgccttcctgagatttatgaggtctggaatgtaactcttcaataggttctgaaacctcggatggtctctcttcggtagcatcctcatcctcaaccttatcctcatcctcttcctcttcttcagaaaaagcatcatccaaatgcaccacttcagacgatgacccagtattcacatgtgtctcatcttgtgttgaactgctctcttgacaatgatatgggtggtgctgcagtacatcctgtaagaaacgttccatcaaactactggtacatatttgacgtctactctgtctggtcaaactcctgtgctgagcactgaacaaatgctttccactgttcttcattacttcctgtatctctgagcttccatcgggaatcattttccttctgcctgaagaactcctttttagtttttcctttagtgagagtctgttccaggttattatactgcacacggcaataactgcaatatccttgtcttttctgcatcttgaataaataactgaagtcagatggctactgtctttgaatactcaagttaaaatttggtctcttttccactaatttacttcacttattaacctggagcagaaaaggtcaggtatttcatcagctgtattagttctggcaagtatctgcgaggcggccgcgggagcccagcgagcggtcctggcgtccctcgggaagaaggcgccccgggcgccc

SEQ ID NO: 18375 - RNA, 6479 nt, Homo sapiens
  source 1..6479: mol_type = other RNA
tgaagtaccagctactcgagaggcttgaggcaggagaatcgcttgaacccaggaagtggaggttgcagtgagcagagatcttgccgctgcattccagcttgagcaacagagcaagatgccatctcaaaaaacaaacaaacacacagaaaagaaattaaatacctgactgcagttctaaataaataaaacaaaatgcagctttcagttctgtgttgatttaatgctttgagtagcaggaaaattgtaaatgtctttgttactgagaaagaatgtaaatcatgcttcagactggttaacgtttttgatgttgttcagatatcaaataccatatgccaattcaggtatttggcacatgggtctggcatccaattgcttatttcatttatgtttttttcccccggaaaaaagtatgtacttattcattcatatgaaacctcctttccccctcattccccgactctatccctcccttcttccctccctccctcactcccctctttccttccttctttcctgtcattcttttgtttctgctatctgcctattttcttttgttttaatgactacaggttctagtacctaaggtaccaatttattggtaagaaaccaaattactttttgtaatgatgccatttaaaagaacaactttcacttactgccttgtgagagaggggaaaaatactatctttttaatgcaagaaaagttcaatataacgtatcaccaaatgtaaatgcaataaagaatgacattgaactctatgttatttgccatttagcttagcagtaccaacatattccagaaactgaaatttctctattgcagataaaaagaataataaacagggaaatctatgccatacatttatgaaacaaatattgttttcttggttttcaacttgcttgcagaaataattattttaatattgtagttcattagccagtatacggtagacatcctctacaggaaaaactaaacaagatgatgattacaaaggagcaggggctgaacttatttgttcaaaatgaacatatgcacaaccttaagcatgctcaagtgtgtgccaggaaaactactacaaagaatcaacggatgtagtgaaatctgcatcatcagtgattgtttctgagcttgggaaaggagtcgttgcctatttggatcctctgcctgaccccagaagaagctgctttgcttcaacatgtccagtggaaatattgcgggaaagtggttacacacttacactaataaatactaggcactgaaatcattctcctgtaataagaatagatgaacatgacaaagaaaatattccgccagaattagagactattccaatgctggctgacttgatggggagaaaggactcattccccttccctccttaccgttccttcctcacctaaattatcactttatatttacaatgaagactgcagtgtttctcccaactttcaaagctgtgtttttttttggggggtggggggcagtgtgtacctcttatgtaaagcaatggtggttttagttttccaccttttggttggcattatctccaaacaaacgctaaaacacgggtaagtggaaccttctgatcctcttgtctttgtaaagaactttagtcagttcaaaatatattgagaaaatgaaaacctatattttaaggaatactgcttttcgtcattttgctaagtgtttagaaagaataatttattgtcataccaataaaagtgagtggaatttgcacttgcattgtcattttcctgcaagaatggaaacgcctatggcacggggagaagcagcatgaggaacgctgaagagatggtgagatggcacatggagtggccttaccacagcagaggtagataaaggtcagaacagactccttcctagccattcccttagaggtcatctgaataaaatcaccctgtgagctcttcctcaggaatcacttgcagcctcaattcctctgcttctcgtccccccagcgccattgaaatctgtattccaccattggttgggataccaaagtgctcatttctacaagtgtttcacagtcaacaattccatgcaattaatgtgtctcccccgagccattcacttcctcagcttgtgtccccagaaaagcaccatgtttccatacactaaaatatgatgcctatgtgtatgtatctgtccacatgtgaatgtatttgcatttgcagaaaaaaaaattttaaaaaaggaacaaaaacgggagaattttgcatttttggtgttttctttttttttgtatttgcgcagaccattttaagattttcagtctcaacaaaacactattaaaacaaagaatctagtaaaatattgtgcatgtactgctaaacaattctagcaattttattaagcaatacctttattatttttgaatattcttaacagactggaacgaaacattttttttcaaaacaaaatatgcatactgtacgcatgtcgcagggttaagtatgatgcagaggttaaagtctgtttgaacaaaaacaaatgcccggggaaatttcatagctataaagttaataactaaattttgttcactaagaggaccttttctatggatttccttcatctctcagtcacactgcaaacttatctgaagtgcacttcccaagtgtagttagagaataggaaggaatgtaaaattttttttttaattatttgttttgtttgtttgtttgtttttttaaaaacagcccttattaactcttccttccactgattctactgtaaactcataaaagccttttatagaaagcaaattcatgtacactcagcaggtgaaatgttcccacaaagaaaataaaatacaaacagtgatcagacctcttttcctcaactacctagagcatgttagagtgataaagtttttgcacgttaataaaaatggctgacctatttattttttaaaaaagaagttgttcctctgtgataatgcagaattgcatacactgtatacctggaataattttaaaccatatgttagggaaatactggaataaaattgtgtatattctgtatattgcaggtgtttgagcatttctagtgtctcttccacaacaataagggaggaaaagaagtccagatatgtgtccgcaatccctttgtttgttccctgtaattacaatggccaaaatgtgctcctatattactgcaacagaacaaaaatcacaatgaaagcccaccttcattgtcaaaagaaaaacttcctcactccccgcatcctgattctagatagctgctcctgtccaactggaccagcaagaaagggctgggccacttggggatgggaactggagcaatacagttcatgatagttttttttaattttttccttttattttgttttcaacataaaaatgtgttaactgtctgattccacctattatggagagcacttgtttgttcagctaaaaaggaactcttgtcaggcccccttggctccgctctgtttctggtttgtgcaacaggggctcagaggcccaccaagcgtgcacacccattcactgtggttacacagacagaagcaagcggatgttgtttgcttaggggacgagaagagggcgagggaaaggaaaggccgggaagggtgttgttggttctgtgggtagaagggagacttagggattttttttatttttatttttttgttgttttcttttttttgtcttttttattttttattctttttttgttgttgttttttgctataccatgaggtcatagcaatcattcctctaatagaagctgacaggacataaagacagaactatctgatgaacacacacaatgactagaaatatatagagagatagagacagtgaaaagacttagtttacctctgagaaaccatcccccaaaataaatcctgtattaacaagtgcaaaaaataaacaaacaaataaacccaaaccaaaacgaaagcaaataaaacctccaaacattaaaacacagtgtataaaatggtgtgagaaatttaaagtcactttccagccttttagtcaataaaaagctgtggttgtgtccttgtttggattcaggcccatctgtttaaattttaccctaaaggccttgcaataagtaattcgagggtaaaagcacccagtttctgttacatgagacagcagttgccatttttcacggcgggccagctgctgctgtggtgacactcgtccttccgttactcctcattggttgagttttcttccagcgtgttgatgcctccaaagctcagtccggctgtgttctgtgctgccgaggctgtgagcactgtgtgtaagagaatcagtacaagaacacacagcttgagtctgctgttgcacagtcttgttgctgatgacactgtgagcgatgtcctgtgacaggagccacttttctctacggtccctttggatgggttatttgatttttcttctctcctgacgtcacagcattctggttcatcattggttagaaaggtttcataaagccctgtacagatgaaactggagaggcctccgtagatgacttcatcattgtcgggcaatataaatggacacctcgtctgaacctccaaacagtattgcttgcaaggaattgtctttctgcagttaaactgtgtgacttcaaaatactgggaacagagccaggctttgtagacaatcttacagtcttcaggacaggatttcaccgagtactcctccgactgtaaatatttgtggagcacgctttcaaactcttcgtatttctcctgagcatggtggtcatagtcctggtaagcctcgacgcactgcctgcaagtggtcatctcgccgccttccttgagcaccacatccagactgcagttcaaagtgttgggactggacaaccccgagaacaactcccaaagtgtgtaggaattacaaaacgaaaggtaaaaatccgacaagttccagagcggagtgggatgcttgctcctcacctcctgcccgtcccccccggccgccccccgactccagttcctggcgcacaccgcgtccgcattctccaccgtgaagcactggcccgaggacgcgccctgggggtaacaagtctccaggcgccacacgggcttggcagagtttcctagaaaaagagccttgccccggtcgtctttgcctcggttgcccttgccgccgccgccgccgccgtctcccggggaggggggcagggtgggggacgaggaggcggagaggagtctgtgtgcctgggcggcgggcgaggactcccccatgctcgccaggagcgcgggccaggagggctcctgctgccgccgctgctgctgctgctgctgccgctgcctctgctgctgctgctgctgctgctgctgccgctgctgctgctggtgctccttgtcccgggcccgggtcagcttggcctcggcgcagaaccacaagtgatcagagagcaggactgtgaaaaacaagagagatgccagagacagtcgccatttctgagccctctcggaatcgatgaacggtttctcgttctctcggggtgctgccaaccagatttttaagccgtcgtcatactgccgacacatccaagcacccctggtcatattttgggaacgcacagccctggccgactccaccgtgagggcgcctgtgccggtgtcaccacaatatgcattgacttaaagggtttaatttccttatcccctcctcccgtttcttctctctcctctctctctttctctctcttcccctctccctctctcctctctctctctctccctctccctctcttttatctctctctgtctcttttgcctacataaatattaccaggctttgaaggaaggtctgacttgcttcctaatcatcagccgaccccatcctctgtagagtgggaaacaataatggagagagagagagagagagagacggaggaggctggtgctggtggccggcggcgaggctgggtgcagggggcgatggtggaggtgacagggtggctggcgcggctccggtcacccaggcattgtcagcgcgcgggtccccatggccccgcggagcccagcccgctctcccctgccaggggcatgccgcgcctccgctgcccactgacggcgcccggagcgcctcccctcctcctcctcctcctcctcttcttctcctcctcttcctcctccttcctttccttctccttcttcttctcctccgcctcccgctcctgctccgcgctggctctcccagagtccggagcctgggctgcctccggcggggcgctccctcccccccaccccccaccccgcgctctaagtgctgccgccgccgccgccgccgccgccgctgccgcagggccgcccgcgggcgccgccgccggggctccgactgctgacgccgcctcccgcggagctccgggccgaatcgcctgggctgggcctcccgagagccacagtcatcttcagtccgcgggctaagttgccgccatcttcgtcctggagaaacactttttt

SEQ ID NO: 18376 - RNA, 3059 nt, Homo sapiens
  source 1..3059: mol_type = other RNA
tgaagtaccagctactcgagagggcgaggcaggacaatcgctcaaacctaggaggtggaggttgcagtgagccaagatcacgccactgcactccagcctgggtaacagagcgagactccatctcaaaataaataaatacataaatgcatatataatctaaacagaaaaatatggaaaaaatagagaaagatgacaaagagatacccttcaaataatgcaccatgcccaaataaattcacaagagaattctataaagcatttaatgaccaaacaacaccaaagtagtgctaattcttccagatacatttattctgtgaagagggctgagacagtttgagggtgagcaaattgattccatatttgtgatgttgaaaatattctgagggcctaagcagatcattctgtggaagggtaatcatgtatactgaggaacatattagtctattctacagttgagaagttgtcactatttctattcaatgtgagttttcccatagacaatgaggactgacttctgggaataggccttcccacaatcagcatatatacaaggtgtctttcctatatggattctgatgcccagtaaagtatacatgctggcagaatgccttcccacagtcactgcatctggagggtttctccccagtgtgtcttctctgatatgtaatcatctgtgatttccagaaaaaagtcattccagactcagcacattcaggggttttctccctaggatgagttttctgatgtataatgagtggagactttccacagaaggcctttccacattcactacattcatagggtttctctccagtatgacctctctgatgtagaatgagatgtgacttcagggaaaaggccctcccacactcagtacactcataaggtttctcccctgtgtgaactctcagatgaataatgaggagtgatttctgggagaaggttttgccacattcaccacactgataaggtttctcccctgtatgaattctctggtgtatgataagaggtgatttctgagagaaggattttccacattcagtacacatataaggtttctctccagtatgaagtctttgatggccagtgaggtgtgacttctgggaaaaggccttcccacagtcagtacacacataaggtttttctcctgtatgaattctttgatgtcctatgaggtgggactgttggcagaaagttttcccacattcaccacacttatagggcttctctccagtatgcgttctctgatgtataatgagctgtgttttccgagggaaggtcttcccacattcagtacattcatagggcttcttcccagtatgagttatctggtgtataaaaaggtgagacatctcacagaaggctttcctgcattcactgcattcaaagggcttctctctggtatgaactctctgatgtataattagatgtgacttctgggagaaagcttttggacactcaaaacactcatagggtttctctccagtatggactctctgatgaacagtgaaaggtgacttccgggagaatgctcttccatacttagtacattcatagggtttctccccagtatgaatcctctgatgcacaatgaggtgtgatttctcactgaaggctttcctacaatctccacatacatatggtttctctccagtatgaattctttgatgtataatgagctgtgacttcttgataaaggctttcccacacatactacaaacattgggtttctctctggcttgaaatttcttatactgaacatgggcttgcttatgactgagaactttttcacattgactatctccatagggctccattccagtatgaatgaagccttccttctcaggcacagaacaggaagcattatacttaggtggtctcccacatctaaatctcttagtggggttctttcttgcatagctcctgttataatttagtaagtctgaattagacttcaagctattttcacatgaatcaaacttatggaatttttgacttaaaggagcaaggtctgtgcaccgattgaacattttcccaaatgcactgtacttggaacccatctcatcagtcaatgtttcacgactgatgactgtgacctgcctcaaaactctgtcttgatttccttgatatctatccatctgattatcaatatgccagatttttaaaacagagtacaatgaattatcctttggggctctttctagtatctccctttgaaataaaagttctccagaaatgatctgctgggaagattcaaggcctttcactctgtctgggtagatccaccttgacaactcactctctatgatccatgggtcctttccatgttccaacttaaagattacatctggttttatacctgaacaccccacggagaccaggtgattataggtctccagcatcacatccctatgcagggtcttctgagcaggattcaactgctgccactcttcctgcgtgaagtccacagccacatcctcaaatgtcactggttcctgggactcaatcattttctgtttctctttggaaagcagttgggggcggggtggggtgcagaagagtcttcggagatcaagctgagttaaccactcttcaacagctggatgtgacaatgtgttgcttgttaattcattgatgacttgtgtttctcatctgactcggtaattccatttccggaacttcgtccccggctctgctctcaagccgggcttggctccccgcctgcccaaatgcgttcaacatcccccgaaaggccatttcccttccagtcttcccggagagatgtcagggtgacgagggagcttatctttcggtggctccgaaacagccacgaagccgagctctaccagtaacaaaaatggcgtcattccgccagcgccaggacctctgtcgctggccgtggtctcgcactgcttctggaggctcccattccagccagaggagaggtgcgtttgggggcccgggggagtcctcgtgatatctccgagtttgggtattcggaattgatcctacgaaagcagtgtgaggcttggaagggccgcgacttgtccgggtgagtg

SEQ ID NO: 18377 - RNA, 2762 nt, Homo sapiens
  source 1..2762: mol_type = other RNA
tgaagtaccagctactcgagagggcgaggcaggacaatcgctcaaacctaggaggtggaggttgcagtgagccaagatcacgccactgcactccagcctgggtaacagagcgagactccatctcaaaataaataaatacataaatgcatatataatctaaacagaaaaatatggaaaaaatagagaaagatgacaaagagatacccttcaaataatgcaccatgcccaaataaattcacaagagaattctataaagcatttaatgaccaaacaacaccaaagtagtgctaattcttccagatacatttattctgtgaagagggctgagacagtttgagggtgagcaaattgattccatatttgtgatgttgaaaatattctgagggcctaagcagatcattctgtggaagggtaatcatgtatactgaggaacatattagtctattctacagttgagaagttgtcactatttctattcaatgtgagttttcccatagacaatgaggactgacttctgggaataggccttcccacaatcagcatatatacaaggtgtctttcctatatggattctgatgcccagtaaagtatacatgctggcagaatgccttcccacagtcactgcatctggagggtttctccccagtgtgtcttctctgatatgtaatcatctgtgatttccagaaaaaagtcattccagactcagcacattcaggggttttctccctaggatgagttttctgatgtataatgagtggagactttccacagaaggcctttccacattcactacattcatagggtttctctccagtatgacctctctgatgtagaatgagatgtgacttcagggaaaaggccctcccacactcagtacactcataaggtttctcccctgtgtgaactctcagatgaataatgaggagtgatttctgggagaaggttttgccacattcaccacactgataaggtttctcccctgtatgaattctctggtgtatgataagaggtgatttctgagagaaggattttccacattcagtacacatataaggtttctctccagtatgaagtctttgatggccagtgaggtgtgacttctgggaaaaggccttcccacagtcagtacacacataaggtttttctcctgtatgaattctttgatgtcctatgaggtgggactgttggcagaaagttttcccacattcaccacacttatagggcttctctccagtatgcgttctctgatgtataatgagctgtgttttccgagggaaggtcttcccacattcagtacattcatagggcttcttcccagtatgagttatctggtgtataaaaaggtgagacatctcacagaaggctttcctgcattcactgcattcaaagggcttctctctggtatgaactctctgatgtataattagatgtgacttctgggagaaagcttttggacactcaaaacactcatagggtttctctccagtatggactctctgatgaacagtgaaaggtgacttccgggagaatgctcttccatacttagtacattcatagggtttctccccagtatgaatcctctgatgcacaatgaggtgtgatttctcactgaaggctttcctacaatctccacatacatatggtttctctccagtatgaattctttgatgtataatgagctgtgacttcttgataaaggctttcccacacatactacaaacattgggtttctctctggcttgaaatttcttatactgaacatgggcttgcttatgactgagaactttttcacattgactatctccatagggctccattccagtatgaatgaagccttccttctcaggcacagaacaggaagcattatacttaggtggtctcccacatctaaatctcttagtggggttctttcttgcatagctcctgttataatttagtaagtctgaattagacttcaagctattttcacatgaatcaaacttatggaatttttgacttaaaggagcaaggtctgtgcaccgattgaacattttcccaaatgcactgtacttggaacccatctcatcagtcaatgtttcacgactgatgactgtgacctgcctcaaaactctgtcttgatttccttgatatctatccatctgattatcaatatgccagatttttaaaacagagtacaatgaattatcctttggggctctttctagtatctccctttgaaataaaagttctccagaaatgatctgctgggaagattcaaggcctttcactctgtctgggtagatccaccttgacaactcactctctatgatccatgggtcctttccatgttccaacttaaagattacatctggttttatacctgaacaccccacggagaccaggtgattataggtctccagcatcacatccctatgcagggtcttctgagcaggattcaactgctgccactcttcctgcgtgaagtccacagccacatcctcaaatgtcactggttcctgggactcaatcattttctgtttctctttggaaagcagttgggggcggggtggggtgcagaagagtcttcggagatcaagctgagttaaccactcttcaacagctggatgtgacaatgtgttgcttgttaattcattgatgacttgtgtttctcatctgactcggtaattccatttccggaacttcgtcccttacagacatcatcaaacaccgcacagatcccccatcaccccacaaactcccatttgcataacccacatactgtt

SEQ ID NO: 18378 - RNA, 2818 nt, Homo sapiens
  source 1..2818: mol_type = other RNA
tgaagtaccagctactcgagagggcgaggcaggacaatcgctcaaacctaggaggtggaggttgcagtgagccaagatcacgccactgcactccagcctgggtaacagagcgagactccatctcaaaataaataaatacataaatgcatatataatctaaacagaaaaatatggaaaaaatagagaaagatgacaaagagatacccttcaaataatgcaccatgcccaaataaattcacaagagaattctataaagcatttaatgaccaaacaacaccaaagtagtgctaattcttccagatacatttattctgtgaagagggctgagacagtttgagggtgagcaaattgattccatatttgtgatgttgaaaatattctgagggcctaagcagatcattctgtggaagggtaatcatgtatactgaggaacatattagtctattctacagttgagaagttgtcactatttctattcaatgtgagttttcccatagacaatgaggactgacttctgggaataggccttcccacaatcagcatatatacaaggtgtctttcctatatggattctgatgcccagtaaagtatacatgctggcagaatgccttcccacagtcactgcatctggagggtttctccccagtgtgtcttctctgatatgtaatcatctgtgatttccagaaaaaagtcattccagactcagcacattcaggggttttctccctaggatgagttttctgatgtataatgagtggagactttccacagaaggcctttccacattcactacattcatagggtttctctccagtatgacctctctgatgtagaatgagatgtgacttcagggaaaaggccctcccacactcagtacactcataaggtttctcccctgtgtgaactctcagatgaataatgaggagtgatttctgggagaaggttttgccacattcaccacactgataaggtttctcccctgtatgaattctctggtgtatgataagaggtgatttctgagagaaggattttccacattcagtacacatataaggtttctctccagtatgaagtctttgatggccagtgaggtgtgacttctgggaaaaggccttcccacagtcagtacacacataaggtttttctcctgtatgaattctttgatgtcctatgaggtgggactgttggcagaaagttttcccacattcaccacacttatagggcttctctccagtatgcgttctctgatgtataatgagctgtgttttccgagggaaggtcttcccacattcagtacattcatagggcttcttcccagtatgagttatctggtgtataaaaaggtgagacatctcacagaaggctttcctgcattcactgcattcaaagggcttctctctggtatgaactctctgatgtataattagatgtgacttctgggagaaagcttttggacactcaaaacactcatagggtttctctccagtatggactctctgatgaacagtgaaaggtgacttccgggagaatgctcttccatacttagtacattcatagggtttctccccagtatgaatcctctgatgcacaatgaggtgtgatttctcactgaaggctttcctacaatctccacatacatatggtttctctccagtatgaattctttgatgtataatgagctgtgacttcttgataaaggctttcccacacatactacaaacattgggtttctctctggcttgaaatttcttatactgaacatgggcttgcttatgactgagaactttttcacattgactatctccatagggctccattccagtatgaatgaagccttccttctcaggcacagaacaggaagcattatacttaggtggtctcccacatctaaatctcttagtggggttctttcttgcatagctcctgttataatttagtaagtctgaattagacttcaagctattttcacatgaatcaaacttatggaatttttgacttaaaggagcaaggtctgtgcaccgattgaacattttcccaaatgcactgtacttggaacccatctcatcagtcaatgtttcacgactgatgactgtgacctgcctcaaaactctgtcttgatttccttgatatctatccatctgattatcaatatgccagatttttaaaacagagtacaatgaattatcctttggggctctttctagtatctccctttgaaataaaagttctccagaaatgatctgctgggaagattcaaggcctttcactctgtctgggtagatccaccttgacaactcactctctatgatccatgggtcctttccatgttccaacttaaagattacatctggttttatacctgaacaccccacggagaccaggtgattataggtctccagcatcacatccctatgcagggtcttctgagcaggattcaactgctgccactcttcctgggactcaatcattttctgtttctctttggaaagcagttgggggcggggtggggtgcagaagagtcttcggagatcaagctgagttaaccactcttcaacagctggatgtgacaatgtgttgcttgttaattcattgatgacttgtgtttctcatctgactcggtaattccatttccggaacttcgtcctctgtcgctggccgtggtctcgcactgcttctggaggctcccattccagccagaggagaggtgcgtttgggggcccgggggagtcctcgtgatatctccgagtttgggtattcggaattgatcctacgaaagcagtgtgaggcttggaagggccgcgacttgtccgggtgagtg

SEQ ID NO: 18379 - RNA, 2019 nt, Homo sapiens
  source 1..2019: mol_type = other RNA
tgaagtaccagctactcgagaggttgaggcaggagaatcgcttgaacccgggaggcagtgggtgtagtgagctgagatctcaccactgcactccagcctagcgacagagcgagaccctgtctcaacaacaacaacaacaaacaaaaaaccccacacattttggaactacaacttacataaaacaaatctctacagagagtgttgaccaaggatgttcaatagtttcatacaggatggaaatgtagccccagaatttcatttttgccacaactattttacccaaactttgttgtactctgtggttccggcaacttggctggttttcctgtagcacggttgtcacaaggaaggcctgttccttgcaggtggactattttgtttgctgatctctgtggcagcccggcaaccctgttgtctaaaatgaactcttggcctctgcagcgccctttgctgtccttgcttcctctgttgttgatcagtctaggtgttctttggatttagtggagcttctgtctctcctctgggtctctcattttaaagtctagcttgagcgtcttcacatggtgctaggtcccaagaagttagctgatgaacttcagctttctcctgattagaggaagagccccaaagcttctatggacactcacttttctcttcttcttcttgcattattatgaggaaatccttaaaggttggggaacttgggcgactttggctaatgaggagctctgtgccttgagccccccaggccatagaatagtaaatagtctgtgcctccagccctgcagtgtgaggttccagtcctgtgggctccacacccatcacctgtatcaggaggctcatgtctcaccctgtcttcttgccagccttgaggatggagtctgagcctccatcgtgcaccacgcagggaggacagtggacttgttctccgtggtcatggcccagcagaggggaagggcagttcagtgagtgctgagggacggttgggagccttgttttgtatcctcatcctcaggaaaaaaacaggagagtgcggtgggcagatgggaggagaccaacgtgcaaactgtcggctcagcagactgtggagtttctgttcttggttatggtcgggggggggcggtctcagaaatcttattcaaaattttgctttcctcccccactggttgtccttttcatagacatctcacccatgatagcagggaatgagtccctctaaactattctctaagaacaataaaaagattatgaaggtgatgatgaggataaagaggatgatgacagacaccatggcatcatgaacccttactgagggcttcctaaaggccaggctctgagctctgtggtctatgcagcttgtttcatttcctctgcgtagtctcccagttattagtgcacatttcattattattttacagactagaaaaggagcaatgcattttcatataacttgtaccagatcatgaagtcaaaaagggtgaagtccagtttgaaccaggcagcctaagtccagacacatggcatttggccagtcctctccctgcatccaacctgccctctcaaatccttgtcactcaggccgatgcccctgctcactgtgcccttccttttgggggttccttgtagaccacagctagaccagtgggtgccacaatcactgtgtcaagtatagaaagggcagctgagatcacatcaaagattccagaaagaattggcacaggatcattcgggatgcatctctcccttgcccctgttcctggctttccttacagctctcgacttcctcaaaggagtcataaattcggaatttggcttctcttcctgttgaggaagctggaaactgtttcaaaaatgctcctcagatgtacctgtggttaagacctctgagctctgctttaaactttttgaagctgggcgcggtggctcacgcctgtaatcccagcactttgggaggctgaggcaggcgaatcacaagttcaggtgttcgagaccagcctggccaacatggtgaaaccccgt

SEQ ID NO: 18380 - RNA, 2022 nt, Homo sapiens
  source 1..2022: mol_type = other RNA
tgaagtaccagctactcgagaggttgaggcaggagaatcgcttgaacccgggaggcagtgggtgtagtgagctgagatctcaccactgcactccagcctagcgacagagcgagaccctgtctcaacaacaacaacaacaaacaaaaaaccccacacattttggaactacaacttacataaaacaaatctctacagagagtgttgaccaaggatgttcaatagtttcatacaggatggaaatgtagccccagaatttcatttttgccacaactattttacccaaactttgttgtactctgtggttccggcaacttggctggttttcctgtagcacggttgtcacaaggaaggcctgttccttgcaggtggactattttgtttgctgatctctgtggcagcccggcaaccctgttgtctaaaatgaactcttggcctctgcagcgccctttgctgtccttgcttcctctgttgttgatcagtctaggtgttctttggatttagtggagcttctgtctctcctctgggtctctcattttaaagtctagcttgagcgtcttcacatggtgctaggtcccaagaagttagctgatgaacttctgcagctttctcctgattagaggaagagccccaaagcttctatggacactcacttttctcttcttcttcttgcattattatgaggaaatccttaaaggttggggaacttgggcgactttggctaatgaggagctctgtgccttgagccccccaggccatagaatagtaaatagtctgtgcctccagccctgcagtgtgaggttccagtcctgtgggctccacacccatcacctgtatcaggaggctcatgtctcaccctgtcttcttgccagccttgaggatggagtctgagcctccatcgtgcaccacgcagggaggacagtggacttgttctccgtggtcatggcccagcagaggggaagggcagttcagtgagtgctgagggacggttgggagccttgttttgtatcctcatcctcaggaaaaaaacaggagagtgcggtgggcagatgggaggagaccaacgtgcaaactgtcggctcagcagactgtggagtttctgttcttggttatggtcgggggggggcggtctcagaaatcttattcaaaattttgctttcctcccccactggttgtccttttcatagacatctcacccatgatagcagggaatgagtccctctaaactattctctaagaacaataaaaagattatgaaggtgatgatgaggataaagaggatgatgacagacaccatggcatcatgaacccttactgagggcttcctaaaggccaggctctgagctctgtggtctatgcagcttgtttcatttcctctgcgtagtctcccagttattagtgcacatttcattattattttacagactagaaaaggagcaatgcattttcatataacttgtaccagatcatgaagtcaaaaagggtgaagtccagtttgaaccaggcagcctaagtccagacacatggcatttggccagtcctctccctgcatccaacctgccctctcaaatccttgtcactcaggccgatgcccctgctcactgtgcccttccttttgggggttccttgtagaccacagctagaccagtgggtgccacaatcactgtgtcaagtatagaaagggcagctgagatcacatcaaagattccagaaagaattggcacaggatcattcgggatgcatctctcccttgcccctgttcctggctttccttacagctctcgacttcctcaaaggagtcataaattcggaatttggcttctcttcctgttgaggaagctggaaactgtttcaaaaatgctcctcagatgtacctgtggttaagacctctgagctctgctttaaactttttgaagctgggcgcggtggctcacgcctgtaatcccagcactttgggaggctgaggcaggcgaatcacaagttcaggtgttcgagaccagcctggccaacatggtgaaaccccgt

SEQ ID NO: 18381 - RNA, 3050 nt, Homo sapiens
  source 1..3050: mol_type = other RNA
tgaagtaccagctactcgagaggttgaggcaggggaatcacttgaatctgggaggcggaggttgcagtgagctgatcacgccactgcactcccgcctggcaacagagcaagactccgtctcaaaaaaaaaaaaaaaacaaaaaaaaccaaaaaaacaaaaccaaccaaaaggcttccacagggaaataactagagaggtggtcttgcagggtctgctgtaattaactggcactatgccaaggaaacaaagctaatgccagtgaaaaatacagtcatttaattctccattttgggtcaatgcaaatgcgtatctcaaaaaaaccaaggttctgaacctctggcaacatcttataattcagtaagatctgctgctggctaaacttagggcatgctagagcagagttgctgggaaaactaagagtaacatcgaactacttgcacatactgagggtacctcaaggcgctggcttccttggagtgcttggacctttaacagaaggtcttagtctaccattgtgtgtgtgcagaaggctgatttgagtttttgcatgattgcacattcatgcacgtagcattactatccatgtgtagcgagactactagatgctagtctgagtctttacctttccatcatctactgtcatgctttcccaagtctgaagatcctgttttccaagatctgtgctcagtaaacaagctttggagtctttaaatgtaaggaataggaaaggtgaagagaggcctggcttaaaatcataacatggagattatggcagtgaatcccattggattgaatggtctgatatggaaagcaggctgtgtagttccactagtccaaaaattctattttttgagacacagtctcgctctgtcacccaggctggagtgaagtggcatgatgtcgactcactgcaacctccgccttccagattcaagcgattctcctgcctcagcttcccaagtagcttggattacagacgcctgccaccacacctggctaatttttgtatttttagtagaaatggggttttgccatgttggccaggctggcctcaaactcctgacctcaagtgatccacccacctcagcctcctaaagtgctgggattacaggtgtgagccactatacctggcctggtccattctttttttttttttttttttttttaagaacaaaactagtttatttggattggggactctgaacagttctgtctctattacccgacttcctcctcccacgacttcggcacctagaggaactttggctccggctgcggtggctcctgcggctctggctccggcggccctggtcccagctgcggtgcctatttcttcctctgcttggtgaattgtgcctctcccgactctttgatgtgcgtttgtgagatttcttccccctatgactactcttttttctctcggattccccatttcttttgtaggtgtggtctggactagggtttctccttccccgctgcctgctgtagtagtggtcgtggtggcccatcttctccctcctctcggagttcttgccaaaggaggagccagtctgatctgaagacaagtagatgtctctattagcttcccagaattcattgttgggatttctgaacacatgaagaaagttgcagtgttttcctcttggacattgttgtatttcaaataaaccacaaatcgccattttccaccgggtcactgggcagaattcacattgcagctgtcgtcctgcataccatcgtccgttaaacagagaaagggctgcttggcattcttcttccgactggtactgaacatatacattgcccctcaggtgaggttccaaattgcagctgaccttgaactgaatcactttccccacgttcttgaactcgggcaacacatcctcatagaaatctaggaactgttggtaggtttcttcctcgctgtactccaggcttgcgtcagggtcatagtcatccctcctgcactgctccattccaaacgttgtaaacatgctcttaataagaagggtaggactagatgttgggaaattatgtttacgtgaacatctgtctccaaatctgcaagctcctgttttactgtagaagggacaattagctcgatccttctccattactctgaaatccacgggtggttctgggttttgccatgtggtactattttctaaatcattttcagcctgatccagcatcttctgcacagcttcctctttttctttcttctcctgttgtttctgctcctcctcttctctctctttcctctgctgttctttccattgttcctttaactttctctcttgttcttctagccattttttagccgcctcttccttttccttctttattctgaattcttcttgtgccttctgctccctcagcaaccactcctcatgtaatctttccctctctctttccaatagcttctcttcttctagttgttgttcttcaataaaagtgtcctcttcctcctcctgtgagagtcctgagtctctcagtcgagcaagttcctgccgacgtttctttcgtttctccttcttcagggcggccctgtactttttgtggcttggtttctctggaaatgtcatcttcttgggaaacgtcatcttctcaagtgcagccatcttgccagcaccgcctgacccctcagacattcttaacgtgatgggaactgtacaaggcagaggctcccatcttcctgtttgagctggacccggactctgcctctgtattggacatcacgattccattctctagagtacattttatttttctcaagaaatacgttaagtccaactgctgaacatacatcttgaatctctgtagctgtaggattttcaacagccttacttatggggattcgccttccctctgcgatggtcttcttattatttaaataagcaggatagatacaaataaacctgtcctggtcggccggggaccgcgcggcagcgcaagccatcttcacaagagtctcaacaacccaggagccgcagggagaaacccggcagaaacccgggaggaacccggctctgagtttccgagacagccc

SEQ ID NO: 18382 - RNA, 1116 nt, Homo sapiens
  source 1..1116: mol_type = other RNA
tgaagtaccagctactcgagagtcatgtattctttttctaaccagtggaggacccagaagaaatggatggcaagctttctcaaaggtccatctggtgagattctggggagcccactcaagtgggaaagaccaaggaagaacaaggcttctattagcaggattatcaggataacactcaggacaataatcagctctgttaatacggtctaagaatacctggtaacattcattttcaacaagttcagtttggtacaaccagtggcctagttctaaactagggaaccactgttgtccacaatcagggcaatgtgaattatctgaaaacatctggacctagaaagacaacacagacagcaatgtgacagcaagagacaacagtgacagagagagacgcccaaacaccagtcctattacaggtttcgtttaccaatttcttagttcaaccaatattatttggagagccaaataaacttggcttgcacctccgtgcaattcttcaagatttcgttgtctatttttcactcaattgcaactcagtctctgaactcagggaccgatccagtttataatgttatcagtcacttactagcagtacagatctcaggatagctccttcaaatcccagcttctcaagaagagatagggctctagtctaaattagttatatttttcttatgcgtcatcagctgctggtggtgtcacacagaggcacttggcttactctgctttgttggtaaggttattgtgtctgcttggtgaaacagaggagctgacaggtccaatgggtcttttgttggcgctggcactcttgccgttgtaacacacgtacccaagtcttaaggccttggcactttatagcaatgtagaggggtcagaaaaacctggcagagtcctcttgatcgtggatccaatgaagtctgtcttgggaggacattaatcaggacccaattgctgtgaagaagctgatgctcagttggctgaagagtctgggaatgcgtcacatacaaattctggcgaagttttaaatcgtaaaactgttagtatcaggagagcccttcgagtattctctccgctccacaccgctcggctgcacccagcggccgccgcggcccgaat

SEQ ID NO: 18383 - RNA, 1038 nt, Homo sapiens
  source 1..1038: mol_type = other RNA
tgaagtaccagctactcgagagtcatgtattctttttctaaccagtggaggacccagaagaaatggatggcaagctttctcaaaggtccatctggtgagattctggggagcccactcaagtgggaaagaccaaggaagaacaaggcttctattagcaggattatcaggataacactcaggacaataatcagctctgttaatacggtctaagaatacctggtaacattcattttcaacaagttcagtttggtacaaccagtggcctagttctaaactagggaaccactgttgtccacaatcagggcaatgtgaattatctgaaaacatctggacctagaaagacaacacagacagcaatgtgacagcaagagacaacagtgacagagagagacgcccaaacaccagtcctattacaggtttcgtttaccaatttcttagttcaaccaatattatttggagagccaaataaacttggcttgcacctccgtgcaattcttcaagatttcgttgtctatttttcactcaattgcaactcagtctctgaactcagggaccgatccagtttataatgttatcagtcacttactagcagtacagatctcaggatagctccttcaaatcccagcttctcaagaagagatagggctctagtctaaattagttatatttttcttatgcgtcatcagctgctggtggtgtcacacagaggcacttggcttactctgctttgttggtaaggttattgtgtctgcttggtgaaacagaggagctgacaggtccaatgggtcttttgttggcgctggcactcttgccgttgtaacacacgtacccaagtcttaaggccttggcactttatagcaatgtagaggggtcagaaaaacctggcagagtcctcttgatcgtggatccaatgaagtctgtcttgggaggacattaatcaggacccaattgctgtgaagaagctgatgctcagttggctgaagagtctgggaatgcgtcacatacataaagtttcaaaaggatataaaattaatgtgt

SEQ ID NO: 18384 - RNA, 1251 nt, Homo sapiens
  source 1..1251: mol_type = other RNA
tgaagtaccagctactcgagagtcatgtattctttttctaaccagtggaggacccagaagaaatggatggcaagctttctcaaaggtccatctggtgagattctggggagcccactcaagtgggaaagaccaaggaagaacaaggcttctattagcaggattatcaggataacactcaggacaataatcagctctgttaatacggtctaagaatacctggtaacattcattttcaacaagttcagtttggtacaaccagtggcctagttctaaactagggaaccactgttgtccacaatcagggcaatgtgaattatctgaaaacatctggacctagaaagacaacacagacagcaatgtgacagcaagagacaacagtgacagagagagacgcccaaacaccagtcctattacaggtttcgtttaccaatttcttagttcaaccaatattatttggagagccaaataaacttggcttgcacctccgtgcaattcttcaagatttcgttgtctatttttcactcaattgcaactcagtctctgaactcagggaccgatccagtttataatgttatcagtcacttactagcagtacagatctcaggatagctccttcaaatcccagcttctcaagaagagatagggctctagtctaaattagttatatttttcttatgcgtcatcagctgctggtggtgtcacacagaggcacttggcttactctgctttgttggtaaggttattgtgtctgcttggtgaaacagaggagctgacaggtccaatgggtcttttgttggcgctggcactcttgccgttgtaacacacgtacccaagtcttaaggccttggcactttatagcaatgtagaggggtcagaaaaacctggcagagtcctcttgatcgtggatccaatgaagtctgtcttgggaggacattaatcaggacccaattgctgtgaagaagctgatgctcagttggctgaagagtctgggaatgcgtcacatacctcgtttactgtttgagtgaggccaggcgtggtggctcacgcctgtaatcccagcactttgggaggctgaggtgggagaatcgcttgaagccaggagttcgagaccaacctgggcaatacagtgagaccctgtcgaaattctggcgaagttttaaatcgtaaaactgttagtatcaggagagcccttcgagtattctctccgctccacaccgctcggctgcacccagcggccgccgcggcccgaat

SEQ ID NO: 18385 - RNA, 2088 nt, Homo sapiens
  source 1..2088: mol_type = other RNA
tgaagtaccagctactcgagagtctgaagcaggagacacacttgaacccgggaggtagaggttgcagtgagccgagatcatgccataatactccagtctgggcaacaagatcataactcagtctcaaaaaaataaataaaaaaaataactgtctgggcgtggtggctcacgcctgtaatcccagcactttgggaggccgaggcgggcgaatcatgaggtcaggagatcgagaccatcctggctaccacaatgaaaccccatctctactaaaaatacaaaaaaattagctgggtgtggtggcaggtgcctgtggtcccagctactcgggaggctgaggcaggagaatggtgtgaacccaggaggcggagcttgcagtgagccgagattgcaccactgcactccagcctgggcgacagagcgaggctccatctcaaaaaaaataaataactatcgtgtactggccttgacaacggtgtgatgaaataattggtacaacaaactccaatgacgtgagtttgcctctgtaacaaaccttcacatgtagccccaaacgtaaagtaaaaaaaaatacataaaaatttttctttaatttacaacagaattttttttaaagtctcataatgatgcagaaatacacgtgtacgagactcgctctgacagctaacacagaactgacaatagtggctcgccagtgaggctggaaggagggtggaggatgtgacagggaaaggagatgccttatggcaaagggtctaagctgcagctttgcttggagttttaccacaaaatatatacatcatgtgatgtttacatataaccatttatattcaataataattgttggggctgggcatggtggcttgcacctgtaatcccaacactcttgggggctgaggcaggcagaccacctgaggttaggagttcgaggccagcctggccaacatggtgaaaccctgtttctactaaaaatacaaaaaaattagccaggcaagccgggcgcggtggctcaagcctgtaatcccagcactttgggaggctgaggtgggaggataacgaggtcaggagattgagaccatcctggctaacacggtgaaaccccgtctctactaaaaacacaaaaaattagctaggcatggtggcgggtgcctgtagtcccagctacttgggaggctgaggcaggagaatggcatgaacccaggaggcagagcttgcagtgagccaagatcataccaaagcactccaccctgggtgacagagtgaaaacatcatctcaaaaaaagaaaaaaaaaattagttggggatggtggcgcgcacctataatcccagctactaggtgggttgagacagagaatcgcttcaacctgggagacagaggttgtagtaagctgagatcatgccactgcactgcagcctgggcaacaaagcaagactccgtttcagaaaataataataataataataataataataataataataaaacgtggaatgagaatacagctttatcctcttagataaaaaagcagtactctccaatattagagaaaaattgcaaccacttttaccaaaaacacctgtttcacaagcctctccacagtaacaccatagtctccgtgagctcgatgtgttaagaatggttgaatgactctcctgctattatttacattgatttcatgttcttaaaataatgaaggaataggccaggaacggtggctcacgcttgtaatcccagcactttaggaagccaaagtaggcggatcgcctgaggtcgggagtttgagaccagcctgatcaacatggagaaacctcgtctctactaaaaatacaaaattagctgagcatggtggcgcatgcttgtaatgccagctactcgggaggctgaggcaggagaatctcttgaacccaggaggcggaggttgcggtgagctgagatcacgccattgcactccagcctgaggaagagccatccctgactcctttgctttcctcttcctcttctgggtttcttcctcacgtaccaagattctttagaagtcaatccgcccgccgcggcgtcaccgtcattccacgggatccgcttcctggtct

SEQ ID NO: 18386 - RNA, 29 nt, Homo sapiens
  source 1..29: mol_type = other RNA
tgaagttacatcatggtcgcttcctagag

SEQ ID NO: 18387 - RNA, 25 nt, Homo sapiens
  source 1..25: mol_type = other RNA
tgaatggtaaagcgatgtcacattg

SEQ ID NO: 18388 - RNA, 46 nt, Homo sapiens
  source 1..46: mol_type = other RNA
tgacaactatggatgagctctcaatatattcttgagttgcatgtct

SEQ ID NO: 18389 - RNA, 885 nt, Homo sapiens
  source 1..885: mol_type = other RNA
tgacagcgccctgcctggctcgaggatgtacgagggatcaaaactcttcaccttgcgcactgtggctgaggctgagctcctcatcccgcccctgatggtgaggcagccaggagggacccaggcagccggtctccctctgtgcgtccctctgggcccctggtgactgcaggtgaccggagctaccaactaagttaatagagatgctccaagtttcacccaaacaggaggcaggtaagcaaggcttggaggcgctagttgaaacaggcctggacggtgacctcgaggaggaggtggagccacgccgggagaggtcccggagagcagcgaggaccggcatctggggtggaggcagcaggcagggtggcaggaggtgcccctgggccacacgagctgtgccgtgcgtttcaaagccatgtgcaacaatgccgggagctgggtagccggcatgcccccgcccagagctgcacaggctgctggtttgtgttgcagaagtgatttccgaagccaagtccatttgagaaacgtgaagagaaacagcatctttacgaccgaatttctggcttgagctgacacactctgcaccccacccaggagctgcggaacgcagtccgtggaaggaaaaactctcttatcaagaacatcttactgtccagtgttcttcctgtggttcgcggtggggctctggctgctggcggccttcagcgtggagcgctgcctctccgacctcttccccgcctgctaccagggctgccggcccagacacgcctcggccgtcctctgcgccctggtgtggaccccgaccctgccggccgtgccgctgcccgccaacgcctgcggcctgctgcgcaacagcgcgtgccccctggtctgcccgcgctaccacgt

SEQ ID NO: 18390 - RNA, 297 nt, Homo sapiens
  source 1..297: mol_type = other RNA
tgacctgggactcggacagctgcttgcactcgttcagctgctcgatccactggtccagctccttggtgaacaccttctcgtccatgatgccacccgccccagccggctgccgctccgcgctgctcccgcgccgccgcccgcacacgggcctacacgcacacgccgccgccggttcctcgtgtacttctggcggctgttgaggctggcgctggcccgctggctctcaccgcagtactcggccgtcggccgctgcgcctcctcctccgctcgctgaggctccagagctcggctctctgt

SEQ ID NO: 18391 - RNA, 1849 nt, Homo sapiens
  source 1..1849: mol_type = other RNA
tgacctttgcctctcccctcaggaaatgctgacttttaacccacacaagcgaatctctgcctttcgagctctgcagcactcttatctacataaggatgaaggtaatccggagtgagcaatggagtggctgccatggaaggaagaaaagctgccatttcccttctggacactgagagggcaatctttgcctttatctctgaggctatggagggtcctcctccatctttctacagagattactttgctgccttaatgacattcccctcccacctctccttttgaggcttctccttctccttcccatttctctacactaaggggtatgttccctcttgtccctttccctacctttatatttggggtccttttttatacaggaaaaacaaaacaaagaaataatggtcttttttttttttttaatgtttcttcctctgtttggctttgccattgtgcgatttggaaaaaccacttggaagaagggactttcctgcaaaaccttaaagactggttaaattacagggcctaggaagtcagtggagccccttgactgacaaagcttagaaaggaactgaaattgcttctttgaatatggattttaggcggggcgtggtggctcacgcctataatcccagcacgttgggaggccaacgcgggtggatcacctgaggtcaggagttcgagaccagcctgactaacatggtgaaaccctgtctctactaaaaatacaaaattagtcaggcgtggtggtgcacacctgtaatcccagctacttgggagactgaggcaggaggatcgcttgaacccgggaggcagaggttgcggtgagccgagatcatgccattgcactccagcctgggcaacagagcaagactctgtgtcaaaaaaaaaaaaagaatatagatttttaaatggcttttacttttatattcgctaaactttctcaaactggatcctgcttattacaggaaagagttcttggttgttttctccttggccctatccctgatttacccttagagccacaccagggtatgttgaggtgatccagtatatggacagaggaagggaaacagctaagaatgactccagcccccatcctatgcactcacagaagcttcccatatcctcttggagagagaggaagaaagtttttccttttattccttatagtctggctcccactaaaatatgtcaaggcataaagtcttgctattccatcaattttagaggatgtgacaaggggcctttcctttttctcaaaccaaaacggttacagaccctagatattccctaagggaggaagagaaagcttagagagagcagaagaaaagtcagaaggatccaaagtctcatagaaaggcactggggttggctctaggatccttctgattccgaaatctcattgctagccaaacaccaaggatctctgtaaagctaaagaagagtccaacaccccctaggattttcagggcttcgtctgaatgcttaagaaacttttctccacacatctggcatgtggggctctggctcttgcagattgcagtgcagaaatcataatcttgttgatacagggttgtgaggttgaataagccacaacaatcaaaacttctttccagttcatcccgagtcttgttgctcatgacccaccaagaagcattgatgacatctgtcatgtagaccacgttgagagcgcaaagcgcattcttggagcaggcaaagccgccacaaaccatctccccagctctggggacccaagtggtcccaaggacttggggggagggtattggggaccgtcttccaggaccccgacagcttctgtctctttaaatcgaggccagccaaacccaat

SEQ ID NO: 18392 - RNA, 2098 nt, Homo sapiens
  source 1..2098: mol_type = other RNA
tgacctttgcctctcccctcaggaaatgctgacttttaacccacacaagcgaatctctgcctttcgagctctgcagcactcttatctacataaggatgaaggtaatccggagtgagcaatggagtggctgccatggaaggaagaaaagctgccatttcccttctggacactgagagggcaatctttgcctttatctctgaggctatggagggtcctcctccatctttctacagagattactttgctgccttaatgacattcccctcccacctctccttttgaggcttctccttctccttcccatttctctacactaaggggtatgttccctcttgtccctttccctacctttatatttggggtccttttttatacaggaaaaacaaaacaaagaaataatggtcttttttttttttttaatgtttcttcctctgtttggctttgccattgtgcgatttggaaaaaccacttggaagaagggactttcctgcaaaaccttaaagactggttaaattacagggcctaggaagtcagtggagccccttgactgacaaagcttagaaaggaactgaaattgcttctttgaatatggattttaggcggggcgtggtggctcacgcctataatcccagcacgttgggaggccaacgcgggtggatcacctgaggtcaggagttcgagaccagcctgactaacatggtgaaaccctgtctctactaaaaatacaaaattagtcaggcgtggtggtgcacacctgtaatcccagctacttgggagactgaggcaggaggatcgcttgaacccgggaggcagaggttgcggtgagccgagatcatgccattgcactccagcctgggcaacagagcaagactctgtgtcaaaaaaaaaaaaagaatatagatttttaaatggcttttacttttatattcgctaaactttctcaaactggatcctgcttattacaggaaagagttcttggttgttttctccttggccctatccctgatttacccttagagccacaccagggtatgttgaggtgatccagtatatggacagaggaagggaaacagctaagaatgactccagcccccatcctatgcactcacagaagcttcccatatcctcttggagagagaggaagaaagtttttccttttattccttatagtctggctcccactaaaatatgtcaaggcataaagtcttgctattccatcaattttagaggatgtgacaaggggcctttcctttttctcaaaccaaaacggttacagaccctagatattccctaagggaggaagagaaagcttagagagagcagaagaaaagtcagaaggatccaaagtctcatagaaaggcactggggttggctctaggatccttctgattccgaaatctcattgctagccaaacaccaaggatctctgtaaagctaaagaagagtccaacaccccctaggattttcagggcttcgtctgaatgcttaagaaacttttctccacacatctggcatgtggggctctggctcttgcagattgcagtgcagaaatcataatcttgttgatacagggttgtgaggttgaataagccacaacaatcaaaacttctttccagttcatcccgagtcttgttgctcatgacccaccaagaagcattgatgacatctgtctgtttgcttcggttaatagccagacatgagcaagagattacaaattggaagatgaagaccaaaccaaggatgatcatgtaaaagaacagcaggacttggtggtggttgacagcacccaccagtccagccactgcaataaggagaaggaagactcccacagcaatgactccgccgatgatgtggatgctggacaccagacccaggcccttgccccaagcagccactccaatgagcaacaagctcaccagcatgtagaccacgttgagagcgcaaagcgcattcttggagcaggcaaagccgccacaaaccatctccccagctctggggacccaagtggtcccaaggacttggggggagggtattggggaccgtcttccaggaccccgacagcttctgtctctttaaatcgaggccagccaaacccaat

SEQ ID NO: 18393 - RNA, 2112 nt, Homo sapiens
  source 1..2112: mol_type = other RNA
tgacctttgcctctcccctcaggaaatgctgacttttaacccacacaagcgaatctctgcctttcgagctctgcagcactcttatctacataaggatgaaggtaatccggagtgagcaatggagtggctgccatggaaggaagaaaagctgccatttcccttctggacactgagagggcaatctttgcctttatctctgaggctatggagggtcctcctccatctttctacagagattactttgctgccttaatgacattcccctcccacctctccttttgaggcttctccttctccttcccatttctctacactaaggggtatgttccctcttgtccctttccctacctttatatttggggtccttttttatacaggaaaaacaaaacaaagaaataatggtcttttttttttttttaatgtttcttcctctgtttggctttgccattgtgcgatttggaaaaaccacttggaagaagggactttcctgcaaaaccttaaagactggttaaattacagggcctaggaagtcagtggagccccttgactgacaaagcttagaaaggaactgaaattgcttctttgaatatggattttaggcggggcgtggtggctcacgcctataatcccagcacgttgggaggccaacgcgggtggatcacctgaggtcaggagttcgagaccagcctgactaacatggtgaaaccctgtctctactaaaaatacaaaattagtcaggcgtggtggtgcacacctgtaatcccagctacttgggagactgaggcaggaggatcgcttgaacccgggaggcagaggttgcggtgagccgagatcatgccattgcactccagcctgggcaacagagcaagactctgtgtcaaaaaaaaaaaaagaatatagatttttaaatggcttttacttttatattcgctaaactttctcaaactggatcctgcttattacaggaaagagttcttggttgttttctccttggccctatccctgatttacccttagagccacaccagggtatgttgaggtgatccagtatatggacagaggaagggaaacagctaagaatgactccagcccccatcctatgcactcacagaagcttcccatatcctcttggagagagaggaagaaagtttttccttttattccttatagtctggctcccactaaaatatgtcaaggcataaagtcttgctattccatcaattttagaggatgtgacaaggggcctttcctttttctcaaaccaaaacggttacagaccctagatattccctaagggaggaagagaaagcttagagagagcagaagaaaagtcagaaggatccaaagtctcatagaaaggcactggggttggctctaggatccttctgattccgaaatctcattgctagccaaacaccaaggatctctgtaaagctaaagaagagtccaacaccccctaggattttcagggcttcgtctgaatgcttaagaaacttttctccacacatctggcatgtggggctctggctcttgcagattgcagtgcagaaatcataatcttgttgatacagggttgtgaggttgaataagccacaacaatcaaaacttctttccagttcatcccgagtcttgttgctcatgacccaccaagaagcattgatgacatctgtctgtttgcttcggttaatagccagacatgagcaagagattacaaattggaagatgaagaccaaaccaaggatgatcatgtaaaagaacagcaggacttggtggtggttgacagcacccaccagtccagccactgcaataaggagaaggaagactcccacagcaatgactccgccgatgatgtggatgctggacaccagacccaggcccttgccccaagcagccactccaatgagcaacaagctcaccagctccaaaacctcaccatgtagaccacgttgagagcgcaaagcgcattcttggagcaggcaaagccgccacaaaccatctccccagctctggggacccaagtggtcccaaggacttggggggagggtattggggaccgtcttccaggaccccgacagcttctgtctctttaaatcgaggccagccaaacccaat

SEQ ID NO: 18394 - RNA, 844 nt, Homo sapiens
  source 1..844: mol_type = other RNA
tgacctttgcctctcccctcagtggaatatcatacatcaatgtgtagaaagtttgttgtgctgggagtgatcagcctccaagcttgtgtggttgctggcagcatttgctttcttgcagactgctggactgagcttcagtttcttgttggctgtcagaggctacctcagttcctagccacctgaccctctcccaagggcagctcacacaacatgacagcttccttcttcaaagccagcaagagaatttctcagcaaggcagatgttgcagtcttacataaggcaaccatgaaaataacatcttgtcacctttgtggcactctactggttagcagtcacaggtctaggccatctcaaggggcagggagtacataaggctgtgaacagcaggtggggatcacagtgaccacctgggagtctatctgccacacctcccagtgcatccaaattctgttgtgcagagggcaagtgaggtctagcataccccccaagaaagcagccatcttctaccatccacccaccagtttgtaaactccagtcaggggtgtaattgaagtgatgcctggtttgggattgagttttcctggagattctggtcctgtaatgagttttttccagctgggattccagttagtgatggacagcatcaagctgtcccttgctcctggccccagaccccacaaggtgcttttcaggctagattcctgagggctgtgtcatcagctgtgccacctcctcctccctaccatgatgaactgttctgggtacttacctgactccagagaaaggtcattaaggtcaaacaatgcaatgtgcatctgctagtgcctcatccgagtgacgctc

SEQ ID NO: 18395 - RNA, 2400 nt, Homo sapiens
  source 1..2400: mol_type = other RNA
tgacctttgcctctcccctcagtggaatatcatacatcaatgtgtagaaagtttgttgtgtggccaggtgcggtggctcacacttgtaatcccagcattttaggaggccaaggcaggctgatcacttgaggtcaggaatttgagaccagcctggccaacatgatgaaaccccgtctctactaaaaatcaaaaaaattagccggaagtactggcacacgtctgtaatcacaactactcggaggctgaggcagaagaactgcttgaacgcaggaggcagaggttgcagtgagctgagatcatgccactgcattccagcctgggccacagagcgagactgtctcaaaacacaaaaaaaacaagtccttacctcatggggttgtagagatgatgcaatgagttttataagtgcatagaatagtgcctagcagagagttaagcattactttagcaataaacaataagcattacttaaaggcaacaggaaggcccaaaggagcatcataagggacctcccaaggccctacagctattaagtctatccagattctctcttttccacactgattcccacctcaaacacactttgctaacctttgtgttggttatctattgctgcataaccttaccagaaacttagcgacttaacacaatacatttaccatctgttcctatgggacagtctgggcacagcttagctggtcctctgcaaggctgcagtcagtgttggtcaggcctggggtctcacctgaaggcttacctgggagtgatcagcctccaagcttgtgtggttgctggcagcatttgctttcttgcagactgctggactgagcttcagtttcttgttggctgtcagaggctacctcagttcctagccacctgaccctctcccaagggcagctcacacaacatgacagcttccttcttcaaagccagcaagagaatttctcagcaaggcagatgttgcagtcttacataaggcaaccatgaaaataacatcttgtcacctttgtggcactctactggttagcagtcacaggtctaggccatctcaaggggcagggagtacataaggctgtgaacagcaggtggggatcacagtgaccacctgggagtctatctgccacacctcccagtgcatccaaattctgttgtgcagagggcaagtgaggtctagcataccccccaagaaagcagccatcttctaccatccacccaccagtttgtaaactccagtcaggggtgtaattgaagtgatgcctggtttgggattgagttttcctggagattctggtcctgtaatgagttttttccagctgggattccagttagtgatggacagcatcaagctgtcccttgctcctggccccagaccccacaaggtgcttttcaggctagattcctgagggctgtgtcatcagctgtgccacctcctcctccctaccatgatgaactgttctgggtacttacctgactccagagaaaggtcattaaggtcaaacaatgcaatgtgcatctgctagtgcctcatccgagtgacgctcaggtgaaggaacagcctgtggccacacgtctaaccaggggatagcctagatcctaaggccaggtctgtctccacaatccaagtgctgatcttcaatggtacatactttttttttttttccttttgagacagtcttgctctgttgcccaggctagagtacagtggcatgatctcagctcactgcaacctccacttcctggaggcaattctcatgcctcagcttctcaagtagctgggattacaggcgtgcgccaccatgcctggctaattgttgtatttttagtagacggggtttcaccatgttcgccaggctggtctcgaactcctaacctcaagtaagccacccacttcggcctcccaaagtgctgggattgtgggcatgagccaccacacccagccatggtacacacttctaataaagcttcctctacatctaagctttctgatttccaccctccaagtacttaaaactgactcgatgtgaagtaatgctatgtgaaatcgacataaaaaagttactgctcccgaagatcctttaatgcaatctccttacccttaattcaatgggcaagagaatcttcaattttcattttctttctcctctctacagtttcttaatcagagtggctatttccataacaataaaaactgcttcttacagaatcctcaggcaaaagaagtgttgtggctttttttcatttttaattcttttagagaattctctagggtctcactgctgcctagactggagtgcgaggccgtgatcatagctcactgcagcctcaaactcctgggctcaagcaattctcccacctcagcctcgcaagtagttaggattccaagcatgcaccaccaccaca

SEQ ID NO: 18396 - RNA, 4341 nt, Homo sapiens
  source 1..4341: mol_type = other RNA
tgacgccccttctgattctgcctctagactggcataagtccacatgagttatgttcttttaaattagaaataacgccatgaagataagtgccaagtgctcttctgttaccagttcatcatggaatttctgttgagggtcatgaaaaacacttggctacttcctccagatcgcacggatgcaaaaaataccttatcatttctttcacatagaaactttaacctttgagctcgcttatgcataaatactccatccaaatgtcctgtttccactgaccggatctcaatagctttctcgccccagcccattatctgattggaatgaatgtaggccacagacgtgggcatttctccccattggagcaccacatccttagttatccggccataggtgtttacatacaccccctcatcctcatagcaaacaagcatttccattccatctgttttaggcaagatgacaatagcatgaggagtgatattgccctgaatatgagatggtatgtagatatcataagagtttcctgaatcaacatcaattacatggaaaccagtgtgtgaaccaaaaataacctttaatctttgaccttcttctaccgtgagatcaactagcagaggcttgtgctggagatctgcaaaagacttaaatgccatgaatttatgatacggtttaggagcccaagcatatatttccacagcattctttaaggcaatcaccaaaaatttgatcctttcatatttaacaactttataatgtatacagccttccaagtccccaacagtgatccagccttgtttcttttctacttctgggtcattatgtagtattctgtttcttaaccatgaaagatagtaaactcgtagcttattcttctttcctgaaattgtcacaaggacattcagtccctctagcacatccatctgctgaaatcgcctccggttgatcagattatagactttgccttgcccacttcggtccaaaagcatcaggccattttcagtccccaccagaaggtttacaccccacagagctgcacaaagtatttctgagttgaatcgtttcttgtattttctgatttctggtgtgtcgctatgaggccgaatgttggttgggtttacatttaccaccgaaatctttcttgcttcattgagtttggcctgttcttgcctaagaagttcgctagtaaacagagctgcggctgatgattcctcatcctcttcatcttcatcagtgggagacgtctggtatactctggggtccacaaagggggtgaaggaggctttggtgctgctccccatgccatattcagtcccagagtccatctcctgggaatgggttgagacgcgccccagtccctcagtcggggttccagctggagaatggctctgctgcaccaggtcagggaggttgatgtggccagcaaagccattgctgtcactgtggccagatcgcttcttctctccagacgtctctctaatcatcaaggttccttctcttgaaatactgccgctgaaactgtccgcatgagaggtctccagcccatgcgtccccaccattcccacattgtactgctcgttgctgcctggagctcctgttggtatcagtctgggtatgtcgctgacagccactgtcccatcatgggtctcgctctctccatcttcctcctcttcctcgctactttctgactcctcactggaggaggagtaatcagtcaccttcttcattgggcggtttgtttcttcaatccggagttctcttagttctttggctaatgccgtcagatcagctggtcgactgggccgggtaatgtccctggattcttctggtttcaccttcgcaggctcatgggggagcacaggtgatccttctgacttactgttggctcgaactctggtgcgttcactggatcctgcttgtgatccaggctgggagcctccttgggagctgggctgggagctaggggtgctggagctggaggaactgccactgctggtcctctgcaaggggctctccaagatgggctcagttctccggagatcagggttgcttgctctgatgggttgagatcctagtctgggtcccagagcactaccattcccaggagaattctttctggctaatgctggggatatagaagttgttctttgaggcacctttggtggaatgtcttcttcctgtcgtaaccaagagcttcggtcaaacttttcaatgcgagtggggagaggaggattttccgaggtgggatctgagttctggcgtggcatctccacgcggtgggaggtcacgttcagagcctcctgaaacccagagaggccctttgtgggctgctcgtgcactgactgggaggcggtcaaggcaggtccctgggattttacagctaccagatgtgggatctccttggcccatgctggcttctcactaggactcattccttctttgtaatggtacagtggcttcttctccacaggcctctgctcctgccgctgatgctgaagggaaactaagtagtctctttcttgctttagctgcctctgcagtctttctgcttgtctctgttcttccaattgtttgcgcttatattccagaagtagagcttgttcatgcagtagctgctgctgcaagatctctaactgtctctgctcctcctctaactgtcgcctgatgtattcctgttcatgctccgcacgcctcctctcctcctcccggcgcatctgctcctcatagtgccggcgctgctccctctcctgctgcttccgcagctccttctctcgcctttgttgctcctccagccgccgcctctgctctttctgctcctcgatgcgcttctgacgctcggccagcagctgccgcttgtgctcctcattctcccgctgctgctgctccagctgctgcctccgtagggcctcagaacgctccttgttggccagctgcagcctcagaaagtccctccgcagcgtcgactcccctggcagattcaggatggagctgggctctcctgagtcattctcctcctcttcttcctcacttccactgtactcatactctgtctcatctttttctcctcgcttcttctttgttctatcaatatggtccttgagttgaatgcggacctgtcgctcattaggttggtctcgtataaatggatgcttcatcaattgttctgttgctggtcgctggctgtgattctttaccaagcagctctcaataaatgactggaatttttttgaccacttcttagacttcagccgaggcgctgggttccgggggatgaggaagagagctctcatggggtgcatgtcacagagagggggagcaccttctgccatttcaatggcggtgatacccaaagaccacaagtcactcttgaaatcatatgtggcatctgggttttcatcacaggcaataacttctggtgccatccagtagggagttccaatgaaagtattcctcctgcccactgttcgatcaagctgagcactgactccaaagtccactagtttaacttctgcattttcagtcagcaagacattttgccctttaatatctcgatgaatcactttatgctggtgcaggtgactcagcccccgtaagatttccctgcagatgtatgcaatccactcctctttcaacgtgttaccttttgtgttcttgatcaggtcggtgacagagccagcaccacaaaactccatcaccaaccaaagttggtcatccatgcctggtgggttctttttgataaaagcaccatagtatgtagcaatattccggtgatgagaatatttcttcaacatgttaatttcttgtttgatttcttcctcttcatcccctgtgacatccataaccttgatggctgcaagctggcccgttttgacatgacgacccttataaacttgcccgtatgttccatttccaacaagttccaccaattcaaagatccctgcggggtccctcagagccgagagatctatttcatccaggcttcgagccggggagtcgctcgccatgtctacttcttcgctggagaaatggaccaaaaccaccccgaagcttttcccttggaaattccaccttggtctatttcactcgcgtcctcatgcgggtgtcgcgccagaggccccgggcccagcctcccccgcccaccccagccccacagcgccggatcccgatcctccgcgcgtcggtccgccgggtccgggagcccagcctgcgcggatctccaagccccgagcagcggtgcgtgtgggctgagcgccccgatcggctaagggcgctggggctgcgtgggtgtatttaaatgggacatgcttctttgcttgtgcgtggatggcggctgcattggctgttat

SEQ ID NO: 18397 - RNA, 4254 nt, Homo sapiens
  source 1..4254: mol_type = other RNA
tgacgccccttctgattctgcctctagactggcataagtccacatgagttatgttcttttaaattagaaataacgccatgaagataagtgccaagtgctcttctgttaccagttcatcatggaatttctgttgagggtcatgaaaaacacttggctacttcctccagatcgcacggatgcaaaaaataccttatcatttctttcacatagaaactttaacctttgagctcgcttatgcataaatactccatccaaatgtcctgtttccactgaccggatctcaatagctttctcgccccagcccattatctgattggaatgaatgtaggccacagacgtgggcatttctccccattggagcaccacatccttagttatccggccataggtgtttacatacaccccctcatcctcatagcaaacaagcatttccattccatctgttttaggcaagatgacaatagcatgaggagtgatattgccctgaatatgagatggtatgtagatatcataagagtttcctgaatcaacatcaattacatggaaaccagtgtgtgaaccaaaaataacctttaatctttgaccttcttctaccgtgagatcaactagcagaggcttgtgctggagatctgcaaaagacttaaatgccatgaatttatgatacggtttaggagcccaagcatatatttccacagcattctttaaggcaatcaccaaaaatttgatcctttcatatttaacaactttataatgtatacagccttccaagtccccaacagtgatccagccttgtttcttttctacttctgggtcattatgtagtattctgtttcttaaccatgaaagatagtaaactcgtagcttattcttctttcctgaaattgtcacaaggacattcagtccctctagcacatccatctgctgaaatcgcctccggttgatcagattatagactttgccttgcccacttcggtccaaaagcatcaggccattttcagtccccaccagaaggtttacaccccacagagctgcacaaagtatttctgagttgaatcgtttcttgtattttctgatttctggtgtgtcgctatgaggccgaatgttggttgggtttacatttaccaccgaaatctttcttgcttcattgagtttggcctgttcttgcctaagaagttcgctagtaaacagagctgcggctgatgattcctcatcctcttcatcttcatcagtgggagacgtctggtatactctggggtccacaaagggggtgaaggaggctttggtgctgctccccatgccatattcagtcccagagtccatctcctgggaatgggttgagacgcgccccagtccctcagtcggggttccagctggagaatggctctgctgcaccaggtcagggaggttgatgtggccagcaaagccattgctgtcactgtggccagatcgcttcttctctccagacgtctctctaatcatcaaggttccttctcttgaaatactgccgctgaaactgtccgcatgagaggtctccagcccatgcgtccccaccattcccacattgtactgctcgttgctgcctggagctcctgttggtatcagtctgggtatgtcgctgacagccactgtcccatcatgggtctcgctctctccatcttcctcctcttcctcgctactttctgactcctcactggaggaggagtaatcagtcaccttcttcattgggcggtttgtttcttcaatccggagttctcttagttctttggctaatgccgtcagatcagctggtcgactgggccgggtaatgtccctggattcttctggtttcaccttcgcaggctcatgggggagcacaggtgatccttctgacttactgttggctcgaactctggtgcgttcactggatcctgcttgtgatccaggctgggagcctccttgggagctgggctgggagctaggggtgctggagctggaggaactgccactgctggtcctctgcaaggggctctccaagatgggctcagttctccggagatcagggttgcttgctctgatgggttgagatcctagtctgggtcccagagcactaccattcccaggagaattctttctggctaatgctggggatatagaagttgttctttgaggcacctttggtggaatgtcttcttcctgtcgtaaccaagagcttcggtcaaacttttcaatgcgagtggggagaggaggattttccgaggtgggatctgagttctggcgtggcatctccacgcggtgggaggtcacgttcagagcctcctgaaacccagagaggccctttgtgggctgctcgtgcactgactgggaggcggtcaaggcaggtccctgggattttacagctaccagatgtgggatctccttggcccatgctggcttctcactaggactcattccttctttgtaatggtacagtggcttcttctccacaggcctctgctcctgccgctgatgctgaagggaaactaagtagtctctttcttgctttagctgcctctgcagtctttctgcttgtctctgttcttccaattgtttgcgcttatattcctgttcatgctccgcacgcctcctctcctcctcccggcgcatctgctcctcatagtgccggcgctgctccctctcctgctgcttccgcagctccttctctcgcctttgttgctcctccagccgccgcctctgctctttctgctcctcgatgcgcttctgacgctcggccagcagctgccgcttgtgctcctcattctcccgctgctgctgctccagctgctgcctccgtagggcctcagaacgctccttgttggccagctgcagcctcagaaagtccctccgcagcgtcgactcccctggcagattcaggatggagctgggctctcctgagtcattctcctcctcttcttcctcacttccactgtactcatactctgtctcatctttttctcctcgcttcttctttgttctatcaatatggtccttgagttgaatgcggacctgtcgctcattaggttggtctcgtataaatggatgcttcatcaattgttctgttgctggtcgctggctgtgattctttaccaagcagctctcaataaatgactggaatttttttgaccacttcttagacttcagccgaggcgctgggttccgggggatgaggaagagagctctcatggggtgcatgtcacagagagggggagcaccttctgccatttcaatggcggtgatacccaaagaccacaagtcactcttgaaatcatatgtggcatctgggttttcatcacaggcaataacttctggtgccatccagtagggagttccaatgaaagtattcctcctgcccactgttcgatcaagctgagcactgactccaaagtccactagtttaacttctgcattttcagtcagcaagacattttgccctttaatatctcgatgaatcactttatgctggtgcaggtgactcagcccccgtaagatttccctgcagatgtatgcaatccactcctctttcaacgtgttaccttttgtgttcttgatcaggtcggtgacagagccagcaccacaaaactccatcaccaaccaaagttggtcatccatgcctggtgggttctttttgataaaagcaccatagtatgtagcaatattccggtgatgagaatatttcttcaacatgttaatttcttgtttgatttcttcctcttcatcccctgtgacatccataaccttgatggctgcaagctggcccgttttgacatgacgacccttataaacttgcccgtatgttccatttccaacaagttccaccaattcaaagatccctgcggggtccctcagagccgagagatctatttcatccaggcttcgagccggggagtcgctcgccatgtctacttcttcgctggagaaatggaccaaaaccaccccgaagcttttcccttggaaattccaccttggtctatttcactcgcgtcctcatgcgggtgtcgcgccagaggccccgggcccagcctcccccgcccaccccagccccacagcgccggatcccgatcctccgcgcgtcggtccgccgggtccgggagcccagcctgcgcggatctccaagccccgagcagcggtgcgtgtgggctgagcgccccgatcggctaagggcgctggggctgcgtgggtgtatttaaatgggacatgcttctttgcttgtgcgtggatggcggctgcattggctgttat

SEQ ID NO: 18398 - RNA, 4506 nt, Homo sapiens
  source 1..4506: mol_type = other RNA
tgacgccccttctgattctgcctctagactggcataagtccacatgagttatgttcttttaaattagaaataacgccatgaagataagtgccaagtgctcttctgttaccagttcatcatggaatttctgttgagggtcatgaaaaacacttggctacttcctccagatcgcacggatgcaaaaaataccttatcatttctttcacatagaaactttaacctttgagctcgcttatgcataaatactccatccaaatgtcctgtttccactgaccggatctcaatagctttctcgccccagcccattatctgattggaatgaatgtaggccacagacgtgggcatttctccccattggagcaccacatccttagttatccggccataggtgtttacatacaccccctcatcctcatagcaaacaagcatttccattccatctgttttaggcaagatgacaatagcatgaggagtgatattgccctgaatatgagatggtatgtagatatcataagagtttcctgaatcaacatcaattacatggaaaccagtgtgtgaaccaaaaataacctttaatctttgaccttcttctaccgtgagatcaactagcagaggcttgtgctggagatctgcaaaagacttaaatgccatgaatttatgatacggtttaggagcccaagcatatatttccacagcattctttaaggcaatcaccaaaaatttgatcctttcatatttaacaactttataatgtatacagccttccaagtccccaacagtgatccagccttgtttcttttctacttctgggtcattatgtagtattctgtttcttaaccatgaaagatagtaaactcgtagcttattcttctttcctgaaattgtcacaaggacattcagtccctctagcacatccatctgctgaaatcgcctccggttgatcagattatagactttgccttgcccacttcggtccaaaagcatcaggccattttcagtccccaccagaaggtttacaccccacagagctgcacaaagtatttctgagttgaatcgtttcttgtattttctgatttctggtgtgtcgctatgaggccgaatgttggttgggtttacatttaccaccgaaatctttcttgcttcattgagtttggcctgttcttgcctaagaagttcgctagtaaacagagctgcggctgatgattcctcatcctcttcatcttcatcagtgggagacgtctggtatactctggggtccacaaagggggtgaaggaggctttggtgctgctccccatgccatattcagtcccagagtccatctcctgggaatgggttgagacgcgccccagtccctcagtcggggttccagctggagaatggctctgctgcaccaggtcagggaggttgatgtggccagcaaagccattgctgtcactgtggccagatcgcttcttctctccagacgtctctctaatcatcaaggttccttctcttgaaatactgccgctgaaactgtccgcatgagaggtctccagcccatgcgtccccaccattcccacattgtactgctcgttgctgcctggagctcctgttggtatcagtctgggtatgtcgctgacagccactgtcccatcatgggtctcgctctctccatcttcctcctcttcctcgctactttctgactcctcactggaggaggagtaatcagtcaccttcttcattgggcggtttgtttcttcaatccggagttctcttagttctttggctaatgccgtcagatcagctggtcgactgggccgggtaatgtccctggattcttctggtttcaccttcgcaggctcatgggggagcacaggtgatccttctgacttactgttggctcgaactctggtgcgttcactggatcctgcttgtgatccaggctgggagcctccttgggagctgggctgggagctaggggtgctggagctggaggaactgccactgctggtcctctgcaaggggctctccaagatgggctcagttctccggagatcagggttgcttgctctgatgggttgagatcctagtctgggtcccagagcactaccattcccaggagaattctttctggctaatgctggggatatagaagttgttctttgaggcacctttggtggaatgtcttcttcctgtcgtaaccaagagcttcggtcaaacttttcaatgcgagtggggagaggaggattttccgaggtgggatctgagttctggcgtggcatctccacgcggtgggaggtcacgttcagagcctcctgaaacccagagaggccctttgtgggctgctcgtgcactgactgggaggcggtcaaggcaggtccctgggattttacagctaccagatgtgggatctggggatcgactggtctgagcatggggggtgttcgagcaggctgaactccactaatgctgaaggactccgaccttgggggcaggttggggtcagatatcctgttggcaaccttgtgaggcatggcaggggaactttgccggttgagccttgaccgttcttctacctccttggcccatgctggcttctcactaggactcattccttctttgtaatggtacagtggcttcttctccacaggcctctgctcctgccgctgatgctgaagggaaactaagtagtctctttcttgctttagctgcctctgcagtctttctgcttgtctctgttcttccaattgtttgcgcttatattccagaagtagagcttgttcatgcagtagctgctgctgcaagatctctaactgtctctgctcctcctctaactgtcgcctgatgtattcctgttcatgctccgcacgcctcctctcctcctcccggcgcatctgctcctcatagtgccggcgctgctccctctcctgctgcttccgcagctccttctctcgcctttgttgctcctccagccgccgcctctgctctttctgctcctcgatgcgcttctgacgctcggccagcagctgccgcttgtgctcctcattctcccgctgctgctgctccagctgctgcctccgtagggcctcagaacgctccttgttggccagctgcagcctcagaaagtccctccgcagcgtcgactcccctggcagattcaggatggagctgggctctcctgagtcattctcctcctcttcttcctcacttccactgtactcatactctgtctcatctttttctcctcgcttcttctttgttctatcaatatggtccttgagttgaatgcggacctgtcgctcattaggttggtctcgtataaatggatgcttcatcaattgttctgttgctggtcgctggctgtgattctttaccaagcagctctcaataaatgactggaatttttttgaccacttcttagacttcagccgaggcgctgggttccgggggatgaggaagagagctctcatggggtgcatgtcacagagagggggagcaccttctgccatttcaatggcggtgatacccaaagaccacaagtcactcttgaaatcatatgtggcatctgggttttcatcacaggcaataacttctggtgccatccagtagggagttccaatgaaagtattcctcctgcccactgttcgatcaagctgagcactgactccaaagtccactagtttaacttctgcattttcagtcagcaagacattttgccctttaatatctcgatgaatcactttatgctggtgcaggtgactcagcccccgtaagatttccctgcagatgtatgcaatccactcctctttcaacgtgttaccttttgtgttcttgatcaggtcggtgacagagccagcaccacaaaactccatcaccaaccaaagttggtcatccatgcctggtgggttctttttgataaaagcaccatagtatgtagcaatattccggtgatgagaatatttcttcaacatgttaatttcttgtttgatttcttcctcttcatcccctgtgacatccataaccttgatggctgcaagctggcccgttttgacatgacgacccttataaacttgcccgtatgttccatttccaacaagttccaccaattcaaagatccctgcggggtccctcagagccgagagatctatttcatccaggcttcgagccggggagtcgctcgccatgtctacttcttcgctggagaaatggaccaaaaccaccccgaagcttttcccttggaaattccaccttggtctatttcactcgcgtcctcatgcgggtgtcgcgccagaggccccgggcccagcctcccccgcccaccccagccccacagcgccggatcccgatcctccgcgcgtcggtccgccgggtccgggagcccagcctgcgcggatctccaagccccgagcagcggtgcgtgtgggctgagcgccccgatcggctaagggcgctggggctgcgtgggtgtatttaaatgggacatgcttctttgcttgtgcgtggatggcggctgcattggctgttat

SEQ ID NO: 18399 - RNA, 4419 nt, Homo sapiens
  source 1..4419: mol_type = other RNA
tgacgccccttctgattctgcctctagactggcataagtccacatgagttatgttcttttaaattagaaataacgccatgaagataagtgccaagtgctcttctgttaccagttcatcatggaatttctgttgagggtcatgaaaaacacttggctacttcctccagatcgcacggatgcaaaaaataccttatcatttctttcacatagaaactttaacctttgagctcgcttatgcataaatactccatccaaatgtcctgtttccactgaccggatctcaatagctttctcgccccagcccattatctgattggaatgaatgtaggccacagacgtgggcatttctccccattggagcaccacatccttagttatccggccataggtgtttacatacaccccctcatcctcatagcaaacaagcatttccattccatctgttttaggcaagatgacaatagcatgaggagtgatattgccctgaatatgagatggtatgtagatatcataagagtttcctgaatcaacatcaattacatggaaaccagtgtgtgaaccaaaaataacctttaatctttgaccttcttctaccgtgagatcaactagcagaggcttgtgctggagatctgcaaaagacttaaatgccatgaatttatgatacggtttaggagcccaagcatatatttccacagcattctttaaggcaatcaccaaaaatttgatcctttcatatttaacaactttataatgtatacagccttccaagtccccaacagtgatccagccttgtttcttttctacttctgggtcattatgtagtattctgtttcttaaccatgaaagatagtaaactcgtagcttattcttctttcctgaaattgtcacaaggacattcagtccctctagcacatccatctgctgaaatcgcctccggttgatcagattatagactttgccttgcccacttcggtccaaaagcatcaggccattttcagtccccaccagaaggtttacaccccacagagctgcacaaagtatttctgagttgaatcgtttcttgtattttctgatttctggtgtgtcgctatgaggccgaatgttggttgggtttacatttaccaccgaaatctttcttgcttcattgagtttggcctgttcttgcctaagaagttcgctagtaaacagagctgcggctgatgattcctcatcctcttcatcttcatcagtgggagacgtctggtatactctggggtccacaaagggggtgaaggaggctttggtgctgctccccatgccatattcagtcccagagtccatctcctgggaatgggttgagacgcgccccagtccctcagtcggggttccagctggagaatggctctgctgcaccaggtcagggaggttgatgtggccagcaaagccattgctgtcactgtggccagatcgcttcttctctccagacgtctctctaatcatcaaggttccttctcttgaaatactgccgctgaaactgtccgcatgagaggtctccagcccatgcgtccccaccattcccacattgtactgctcgttgctgcctggagctcctgttggtatcagtctgggtatgtcgctgacagccactgtcccatcatgggtctcgctctctccatcttcctcctcttcctcgctactttctgactcctcactggaggaggagtaatcagtcaccttcttcattgggcggtttgtttcttcaatccggagttctcttagttctttggctaatgccgtcagatcagctggtcgactgggccgggtaatgtccctggattcttctggtttcaccttcgcaggctcatgggggagcacaggtgatccttctgacttactgttggctcgaactctggtgcgttcactggatcctgcttgtgatccaggctgggagcctccttgggagctgggctgggagctaggggtgctggagctggaggaactgccactgctggtcctctgcaaggggctctccaagatgggctcagttctccggagatcagggttgcttgctctgatgggttgagatcctagtctgggtcccagagcactaccattcccaggagaattctttctggctaatgctggggatatagaagttgttctttgaggcacctttggtggaatgtcttcttcctgtcgtaaccaagagcttcggtcaaacttttcaatgcgagtggggagaggaggattttccgaggtgggatctgagttctggcgtggcatctccacgcggtgggaggtcacgttcagagcctcctgaaacccagagaggccctttgtgggctgctcgtgcactgactgggaggcggtcaaggcaggtccctgggattttacagctaccagatgtgggatctggggatcgactggtctgagcatggggggtgttcgagcaggctgaactccactaatgctgaaggactccgaccttgggggcaggttggggtcagatatcctgttggcaaccttgtgaggcatggcaggggaactttgccggttgagccttgaccgttcttctacctccttggcccatgctggcttctcactaggactcattccttctttgtaatggtacagtggcttcttctccacaggcctctgctcctgccgctgatgctgaagggaaactaagtagtctctttcttgctttagctgcctctgcagtctttctgcttgtctctgttcttccaattgtttgcgcttatattcctgttcatgctccgcacgcctcctctcctcctcccggcgcatctgctcctcatagtgccggcgctgctccctctcctgctgcttccgcagctccttctctcgcctttgttgctcctccagccgccgcctctgctctttctgctcctcgatgcgcttctgacgctcggccagcagctgccgcttgtgctcctcattctcccgctgctgctgctccagctgctgcctccgtagggcctcagaacgctccttgttggccagctgcagcctcagaaagtccctccgcagcgtcgactcccctggcagattcaggatggagctgggctctcctgagtcattctcctcctcttcttcctcacttccactgtactcatactctgtctcatctttttctcctcgcttcttctttgttctatcaatatggtccttgagttgaatgcggacctgtcgctcattaggttggtctcgtataaatggatgcttcatcaattgttctgttgctggtcgctggctgtgattctttaccaagcagctctcaataaatgactggaatttttttgaccacttcttagacttcagccgaggcgctgggttccgggggatgaggaagagagctctcatggggtgcatgtcacagagagggggagcaccttctgccatttcaatggcggtgatacccaaagaccacaagtcactcttgaaatcatatgtggcatctgggttttcatcacaggcaataacttctggtgccatccagtagggagttccaatgaaagtattcctcctgcccactgttcgatcaagctgagcactgactccaaagtccactagtttaacttctgcattttcagtcagcaagacattttgccctttaatatctcgatgaatcactttatgctggtgcaggtgactcagcccccgtaagatttccctgcagatgtatgcaatccactcctctttcaacgtgttaccttttgtgttcttgatcaggtcggtgacagagccagcaccacaaaactccatcaccaaccaaagttggtcatccatgcctggtgggttctttttgataaaagcaccatagtatgtagcaatattccggtgatgagaatatttcttcaacatgttaatttcttgtttgatttcttcctcttcatcccctgtgacatccataaccttgatggctgcaagctggcccgttttgacatgacgacccttataaacttgcccgtatgttccatttccaacaagttccaccaattcaaagatccctgcggggtccctcagagccgagagatctatttcatccaggcttcgagccggggagtcgctcgccatgtctacttcttcgctggagaaatggaccaaaaccaccccgaagcttttcccttggaaattccaccttggtctatttcactcgcgtcctcatgcgggtgtcgcgccagaggccccgggcccagcctcccccgcccaccccagccccacagcgccggatcccgatcctccgcgcgtcggtccgccgggtccgggagcccagcctgcgcggatctccaagccccgagcagcggtgcgtgtgggctgagcgccccgatcggctaagggcgctggggctgcgtgggtgtatttaaatgggacatgcttctttgcttgtgcgtggatggcggctgcattggctgttat

SEQ ID NO: 18400 - RNA, 4365 nt, Homo sapiens
  source 1..4365: mol_type = other RNA
tgacgccccttctgattctgcctctagactggcataagtccacatgagttatgttcttttaaattagaaataacgccatgaagataagtgccaagtgctcttctgttaccagttcatcatggaatttctgttgagggtcatgaaaaacacttggctacttcctccagatcgcacggatgcaaaaaataccttatcatttctttcacatagaaactttaacctttgagctcgcttatgcataaatactccatccaaatgtcctgtttccactgaccggatctcaatagctttctcgccccagcccattatctgattggaatgaatgtaggccacagacgtgggcatttctccccattggagcaccacatccttagttatccggccataggtgtttacatacaccccctcatcctcatagcaaacaagcatttccattccatctgttttaggcaagatgacaatagcatgaggagtgatattgccctgaatatgagatggtatgtagatatcataagagtttcctgaatcaacatcaattacatggaaaccagtgtgtgaaccaaaaataacctttaatctttgaccttcttctaccgtgagatcaactagcagaggcttgtgctggagatctgcaaaagacttaaatgccatgaatttatgatacggtttaggagcccaagcatatatttccacagcattctttaaggcaatcaccaaaaatttgatcctttcatatttaacaactttataatgtatacagccttccaagtccccaacagtgatccagccttgtttcttttctacttctgggtcattatgtagtattctgtttcttaaccatgaaagatagtaaactcgtagcttattcttctttcctgaaattgtcacaaggacattcagtccctctagcacatccatctgctgaaatcgcctccggttgatcagattatagactttgccttgcccacttcggtccaaaagcatcaggccattttcagtccccaccagaaggtttacaccccacagagctgcacaaagtatttctgagttgaatcgtttcttgtattttctgatttctggtgtgtcgctatgaggccgaatgttggttgggtttacatttaccaccgaaatctttcttgcttcattgagtttggcctgttcttgcctaagaagttcgctagtaaacagagctgcggctgatgattcctcatcctcttcatcttcatcagtgggagacgtctggtatactctggggtccacaaagggggtgaaggaggctttggtgctgctccccatgccatattcagtcccagagtccatctcctgggaatgggttgagacgcgccccagtccctcagtcggggttccagctggagaatggctctgctgcaccaggtcagggaggttgatgtggccagcaaagccattgctgtcactgtggccagatcgcttcttctctccagacgtctctctaatcatcaaggttccttctcttgaaatactgccgctgaaactgtccgcatgagaggtctccagcccatgcgtccccaccattcccacattgtactgctcgttgctgcctggagctcctgttggtatcagtctgggtatgtcgctgacagccactgtcccatcatgggtctcgctctctccatcttcctcctcttcctcgctactttctgactcctcactggaggaggagtaatcagtcaccttcttcattgggcggtttgtttcttcaatccggagttctcttagttctttggctaatgccgtcagatcctcatctatagcttttttgtagctagctggtcgactgggccgggtaatgtccctggattcttctggtttcaccttcgcaggctcatgggggagcacaggtgatccttctgacttactgttggctcgaactctggtgcgttcactggatcctgcttgtgatccaggctgggagcctccttgggagctgggctgggagctaggggtgctggagctggaggaactgccactgctggtcctctgcaaggggctctccaagatgggctcagttctccggagatcagggttgcttgctctgatgggttgagatcctagtctgggtcccagagcactaccattcccaggagaattctttctggctaatgctggggatatagaagttgttctttgaggcacctttggtggaatgtcttcttcctgtcgtaaccaagagcttcggtcaaacttttcaatgcgagtggggagaggaggattttccgaggtgggatctgagttctggcgtggcatctccacgcggtgggaggtcacgttcagagcctcctgaaacccagagaggccctttgtgggctgctcgtgcactgactgggaggcggtcaaggcaggtccctgggattttacagctaccagatgtgggatctccttggcccatgctggcttctcactaggactcattccttctttgtaatggtacagtggcttcttctccacaggcctctgctcctgccgctgatgctgaagggaaactaagtagtctctttcttgctttagctgcctctgcagtctttctgcttgtctctgttcttccaattgtttgcgcttatattccagaagtagagcttgttcatgcagtagctgctgctgcaagatctctaactgtctctgctcctcctctaactgtcgcctgatgtattcctgttcatgctccgcacgcctcctctcctcctcccggcgcatctgctcctcatagtgccggcgctgctccctctcctgctgcttccgcagctccttctctcgcctttgttgctcctccagccgccgcctctgctctttctgctcctcgatgcgcttctgacgctcggccagcagctgccgcttgtgctcctcattctcccgctgctgctgctccagctgctgcctccgtagggcctcagaacgctccttgttggccagctgcagcctcagaaagtccctccgcagcgtcgactcccctggcagattcaggatggagctgggctctcctgagtcattctcctcctcttcttcctcacttccactgtactcatactctgtctcatctttttctcctcgcttcttctttgttctatcaatatggtccttgagttgaatgcggacctgtcgctcattaggttggtctcgtataaatggatgcttcatcaattgttctgttgctggtcgctggctgtgattctttaccaagcagctctcaataaatgactggaatttttttgaccacttcttagacttcagccgaggcgctgggttccgggggatgaggaagagagctctcatggggtgcatgtcacagagagggggagcaccttctgccatttcaatggcggtgatacccaaagaccacaagtcactcttgaaatcatatgtggcatctgggttttcatcacaggcaataacttctggtgccatccagtagggagttccaatgaaagtattcctcctgcccactgttcgatcaagctgagcactgactccaaagtccactagtttaacttctgcattttcagtcagcaagacattttgccctttaatatctcgatgaatcactttatgctggtgcaggtgactcagcccccgtaagatttccctgcagatgtatgcaatccactcctctttcaacgtgttaccttttgtgttcttgatcaggtcggtgacagagccagcaccacaaaactccatcaccaaccaaagttggtcatccatgcctggtgggttctttttgataaaagcaccatagtatgtagcaatattccggtgatgagaatatttcttcaacatgttaatttcttgtttgatttcttcctcttcatcccctgtgacatccataaccttgatggctgcaagctggcccgttttgacatgacgacccttataaacttgcccgtatgttccatttccaacaagttccaccaattcaaagatccctgcggggtccctcagagccgagagatctatttcatccaggcttcgagccggggagtcgctcgccatgtctacttcttcgctggagaaatggaccaaaaccaccccgaagcttttcccttggaaattccaccttggtctatttcactcgcgtcctcatgcgggtgtcgcgccagaggccccgggcccagcctcccccgcccaccccagccccacagcgccggatcccgatcctccgcgcgtcggtccgccgggtccgggagcccagcctgcgcggatctccaagccccgagcagcggtgcgtgtgggctgagcgccccgatcggctaagggcgctggggctgcgtgggtgtatttaaatgggacatgcttctttgcttgtgcgtggatggcggctgcattggctgttat

SEQ ID NO: 18401 - RNA, 4278 nt, Homo sapiens
  source 1..4278: mol_type = other RNA
tgacgccccttctgattctgcctctagactggcataagtccacatgagttatgttcttttaaattagaaataacgccatgaagataagtgccaagtgctcttctgttaccagttcatcatggaatttctgttgagggtcatgaaaaacacttggctacttcctccagatcgcacggatgcaaaaaataccttatcatttctttcacatagaaactttaacctttgagctcgcttatgcataaatactccatccaaatgtcctgtttccactgaccggatctcaatagctttctcgccccagcccattatctgattggaatgaatgtaggccacagacgtgggcatttctccccattggagcaccacatccttagttatccggccataggtgtttacatacaccccctcatcctcatagcaaacaagcatttccattccatctgttttaggcaagatgacaatagcatgaggagtgatattgccctgaatatgagatggtatgtagatatcataagagtttcctgaatcaacatcaattacatggaaaccagtgtgtgaaccaaaaataacctttaatctttgaccttcttctaccgtgagatcaactagcagaggcttgtgctggagatctgcaaaagacttaaatgccatgaatttatgatacggtttaggagcccaagcatatatttccacagcattctttaaggcaatcaccaaaaatttgatcctttcatatttaacaactttataatgtatacagccttccaagtccccaacagtgatccagccttgtttcttttctacttctgggtcattatgtagtattctgtttcttaaccatgaaagatagtaaactcgtagcttattcttctttcctgaaattgtcacaaggacattcagtccctctagcacatccatctgctgaaatcgcctccggttgatcagattatagactttgccttgcccacttcggtccaaaagcatcaggccattttcagtccccaccagaaggtttacaccccacagagctgcacaaagtatttctgagttgaatcgtttcttgtattttctgatttctggtgtgtcgctatgaggccgaatgttggttgggtttacatttaccaccgaaatctttcttgcttcattgagtttggcctgttcttgcctaagaagttcgctagtaaacagagctgcggctgatgattcctcatcctcttcatcttcatcagtgggagacgtctggtatactctggggtccacaaagggggtgaaggaggctttggtgctgctccccatgccatattcagtcccagagtccatctcctgggaatgggttgagacgcgccccagtccctcagtcggggttccagctggagaatggctctgctgcaccaggtcagggaggttgatgtggccagcaaagccattgctgtcactgtggccagatcgcttcttctctccagacgtctctctaatcatcaaggttccttctcttgaaatactgccgctgaaactgtccgcatgagaggtctccagcccatgcgtccccaccattcccacattgtactgctcgttgctgcctggagctcctgttggtatcagtctgggtatgtcgctgacagccactgtcccatcatgggtctcgctctctccatcttcctcctcttcctcgctactttctgactcctcactggaggaggagtaatcagtcaccttcttcattgggcggtttgtttcttcaatccggagttctcttagttctttggctaatgccgtcagatcctcatctatagcttttttgtagctagctggtcgactgggccgggtaatgtccctggattcttctggtttcaccttcgcaggctcatgggggagcacaggtgatccttctgacttactgttggctcgaactctggtgcgttcactggatcctgcttgtgatccaggctgggagcctccttgggagctgggctgggagctaggggtgctggagctggaggaactgccactgctggtcctctgcaaggggctctccaagatgggctcagttctccggagatcagggttgcttgctctgatgggttgagatcctagtctgggtcccagagcactaccattcccaggagaattctttctggctaatgctggggatatagaagttgttctttgaggcacctttggtggaatgtcttcttcctgtcgtaaccaagagcttcggtcaaacttttcaatgcgagtggggagaggaggattttccgaggtgggatctgagttctggcgtggcatctccacgcggtgggaggtcacgttcagagcctcctgaaacccagagaggccctttgtgggctgctcgtgcactgactgggaggcggtcaaggcaggtccctgggattttacagctaccagatgtgggatctccttggcccatgctggcttctcactaggactcattccttctttgtaatggtacagtggcttcttctccacaggcctctgctcctgccgctgatgctgaagggaaactaagtagtctctttcttgctttagctgcctctgcagtctttctgcttgtctctgttcttccaattgtttgcgcttatattcctgttcatgctccgcacgcctcctctcctcctcccggcgcatctgctcctcatagtgccggcgctgctccctctcctgctgcttccgcagctccttctctcgcctttgttgctcctccagccgccgcctctgctctttctgctcctcgatgcgcttctgacgctcggccagcagctgccgcttgtgctcctcattctcccgctgctgctgctccagctgctgcctccgtagggcctcagaacgctccttgttggccagctgcagcctcagaaagtccctccgcagcgtcgactcccctggcagattcaggatggagctgggctctcctgagtcattctcctcctcttcttcctcacttccactgtactcatactctgtctcatctttttctcctcgcttcttctttgttctatcaatatggtccttgagttgaatgcggacctgtcgctcattaggttggtctcgtataaatggatgcttcatcaattgttctgttgctggtcgctggctgtgattctttaccaagcagctctcaataaatgactggaatttttttgaccacttcttagacttcagccgaggcgctgggttccgggggatgaggaagagagctctcatggggtgcatgtcacagagagggggagcaccttctgccatttcaatggcggtgatacccaaagaccacaagtcactcttgaaatcatatgtggcatctgggttttcatcacaggcaataacttctggtgccatccagtagggagttccaatgaaagtattcctcctgcccactgttcgatcaagctgagcactgactccaaagtccactagtttaacttctgcattttcagtcagcaagacattttgccctttaatatctcgatgaatcactttatgctggtgcaggtgactcagcccccgtaagatttccctgcagatgtatgcaatccactcctctttcaacgtgttaccttttgtgttcttgatcaggtcggtgacagagccagcaccacaaaactccatcaccaaccaaagttggtcatccatgcctggtgggttctttttgataaaagcaccatagtatgtagcaatattccggtgatgagaatatttcttcaacatgttaatttcttgtttgatttcttcctcttcatcccctgtgacatccataaccttgatggctgcaagctggcccgttttgacatgacgacccttataaacttgcccgtatgttccatttccaacaagttccaccaattcaaagatccctgcggggtccctcagagccgagagatctatttcatccaggcttcgagccggggagtcgctcgccatgtctacttcttcgctggagaaatggaccaaaaccaccccgaagcttttcccttggaaattccaccttggtctatttcactcgcgtcctcatgcgggtgtcgcgccagaggccccgggcccagcctcccccgcccaccccagccccacagcgccggatcccgatcctccgcgcgtcggtccgccgggtccgggagcccagcctgcgcggatctccaagccccgagcagcggtgcgtgtgggctgagcgccccgatcggctaagggcgctggggctgcgtgggtgtatttaaatgggacatgcttctttgcttgtgcgtggatggcggctgcattggctgttat

SEQ ID NO: 18402 - RNA, 4530 nt, Homo sapiens
  source 1..4530: mol_type = other RNA
tgacgccccttctgattctgcctctagactggcataagtccacatgagttatgttcttttaaattagaaataacgccatgaagataagtgccaagtgctcttctgttaccagttcatcatggaatttctgttgagggtcatgaaaaacacttggctacttcctccagatcgcacggatgcaaaaaataccttatcatttctttcacatagaaactttaacctttgagctcgcttatgcataaatactccatccaaatgtcctgtttccactgaccggatctcaatagctttctcgccccagcccattatctgattggaatgaatgtaggccacagacgtgggcatttctccccattggagcaccacatccttagttatccggccataggtgtttacatacaccccctcatcctcatagcaaacaagcatttccattccatctgttttaggcaagatgacaatagcatgaggagtgatattgccctgaatatgagatggtatgtagatatcataagagtttcctgaatcaacatcaattacatggaaaccagtgtgtgaaccaaaaataacctttaatctttgaccttcttctaccgtgagatcaactagcagaggcttgtgctggagatctgcaaaagacttaaatgccatgaatttatgatacggtttaggagcccaagcatatatttccacagcattctttaaggcaatcaccaaaaatttgatcctttcatatttaacaactttataatgtatacagccttccaagtccccaacagtgatccagccttgtttcttttctacttctgggtcattatgtagtattctgtttcttaaccatgaaagatagtaaactcgtagcttattcttctttcctgaaattgtcacaaggacattcagtccctctagcacatccatctgctgaaatcgcctccggttgatcagattatagactttgccttgcccacttcggtccaaaagcatcaggccattttcagtccccaccagaaggtttacaccccacagagctgcacaaagtatttctgagttgaatcgtttcttgtattttctgatttctggtgtgtcgctatgaggccgaatgttggttgggtttacatttaccaccgaaatctttcttgcttcattgagtttggcctgttcttgcctaagaagttcgctagtaaacagagctgcggctgatgattcctcatcctcttcatcttcatcagtgggagacgtctggtatactctggggtccacaaagggggtgaaggaggctttggtgctgctccccatgccatattcagtcccagagtccatctcctgggaatgggttgagacgcgccccagtccctcagtcggggttccagctggagaatggctctgctgcaccaggtcagggaggttgatgtggccagcaaagccattgctgtcactgtggccagatcgcttcttctctccagacgtctctctaatcatcaaggttccttctcttgaaatactgccgctgaaactgtccgcatgagaggtctccagcccatgcgtccccaccattcccacattgtactgctcgttgctgcctggagctcctgttggtatcagtctgggtatgtcgctgacagccactgtcccatcatgggtctcgctctctccatcttcctcctcttcctcgctactttctgactcctcactggaggaggagtaatcagtcaccttcttcattgggcggtttgtttcttcaatccggagttctcttagttctttggctaatgccgtcagatcctcatctatagcttttttgtagctagctggtcgactgggccgggtaatgtccctggattcttctggtttcaccttcgcaggctcatgggggagcacaggtgatccttctgacttactgttggctcgaactctggtgcgttcactggatcctgcttgtgatccaggctgggagcctccttgggagctgggctgggagctaggggtgctggagctggaggaactgccactgctggtcctctgcaaggggctctccaagatgggctcagttctccggagatcagggttgcttgctctgatgggttgagatcctagtctgggtcccagagcactaccattcccaggagaattctttctggctaatgctggggatatagaagttgttctttgaggcacctttggtggaatgtcttcttcctgtcgtaaccaagagcttcggtcaaacttttcaatgcgagtggggagaggaggattttccgaggtgggatctgagttctggcgtggcatctccacgcggtgggaggtcacgttcagagcctcctgaaacccagagaggccctttgtgggctgctcgtgcactgactgggaggcggtcaaggcaggtccctgggattttacagctaccagatgtgggatctggggatcgactggtctgagcatggggggtgttcgagcaggctgaactccactaatgctgaaggactccgaccttgggggcaggttggggtcagatatcctgttggcaaccttgtgaggcatggcaggggaactttgccggttgagccttgaccgttcttctacctccttggcccatgctggcttctcactaggactcattccttctttgtaatggtacagtggcttcttctccacaggcctctgctcctgccgctgatgctgaagggaaactaagtagtctctttcttgctttagctgcctctgcagtctttctgcttgtctctgttcttccaattgtttgcgcttatattccagaagtagagcttgttcatgcagtagctgctgctgcaagatctctaactgtctctgctcctcctctaactgtcgcctgatgtattcctgttcatgctccgcacgcctcctctcctcctcccggcgcatctgctcctcatagtgccggcgctgctccctctcctgctgcttccgcagctccttctctcgcctttgttgctcctccagccgccgcctctgctctttctgctcctcgatgcgcttctgacgctcggccagcagctgccgcttgtgctcctcattctcccgctgctgctgctccagctgctgcctccgtagggcctcagaacgctccttgttggccagctgcagcctcagaaagtccctccgcagcgtcgactcccctggcagattcaggatggagctgggctctcctgagtcattctcctcctcttcttcctcacttccactgtactcatactctgtctcatctttttctcctcgcttcttctttgttctatcaatatggtccttgagttgaatgcggacctgtcgctcattaggttggtctcgtataaatggatgcttcatcaattgttctgttgctggtcgctggctgtgattctttaccaagcagctctcaataaatgactggaatttttttgaccacttcttagacttcagccgaggcgctgggttccgggggatgaggaagagagctctcatggggtgcatgtcacagagagggggagcaccttctgccatttcaatggcggtgatacccaaagaccacaagtcactcttgaaatcatatgtggcatctgggttttcatcacaggcaataacttctggtgccatccagtagggagttccaatgaaagtattcctcctgcccactgttcgatcaagctgagcactgactccaaagtccactagtttaacttctgcattttcagtcagcaagacattttgccctttaatatctcgatgaatcactttatgctggtgcaggtgactcagcccccgtaagatttccctgcagatgtatgcaatccactcctctttcaacgtgttaccttttgtgttcttgatcaggtcggtgacagagccagcaccacaaaactccatcaccaaccaaagttggtcatccatgcctggtgggttctttttgataaaagcaccatagtatgtagcaatattccggtgatgagaatatttcttcaacatgttaatttcttgtttgatttcttcctcttcatcccctgtgacatccataaccttgatggctgcaagctggcccgttttgacatgacgacccttataaacttgcccgtatgttccatttccaacaagttccaccaattcaaagatccctgcggggtccctcagagccgagagatctatttcatccaggcttcgagccggggagtcgctcgccatgtctacttcttcgctggagaaatggaccaaaaccaccccgaagcttttcccttggaaattccaccttggtctatttcactcgcgtcctcatgcgggtgtcgcgccagaggccccgggcccagcctcccccgcccaccccagccccacagcgccggatcccgatcctccgcgcgtcggtccgccgggtccgggagcccagcctgcgcggatctccaagccccgagcagcggtgcgtgtgggctgagcgccccgatcggctaagggcgctggggctgcgtgggtgtatttaaatgggacatgcttctttgcttgtgcgtggatggcggctgcattggctgttat

SEQ ID NO: 18403 - RNA, 4443 nt, Homo sapiens
  source 1..4443: mol_type = other RNA
tgacgccccttctgattctgcctctagactggcataagtccacatgagttatgttcttttaaattagaaataacgccatgaagataagtgccaagtgctcttctgttaccagttcatcatggaatttctgttgagggtcatgaaaaacacttggctacttcctccagatcgcacggatgcaaaaaataccttatcatttctttcacatagaaactttaacctttgagctcgcttatgcataaatactccatccaaatgtcctgtttccactgaccggatctcaatagctttctcgccccagcccattatctgattggaatgaatgtaggccacagacgtgggcatttctccccattggagcaccacatccttagttatccggccataggtgtttacatacaccccctcatcctcatagcaaacaagcatttccattccatctgttttaggcaagatgacaatagcatgaggagtgatattgccctgaatatgagatggtatgtagatatcataagagtttcctgaatcaacatcaattacatggaaaccagtgtgtgaaccaaaaataacctttaatctttgaccttcttctaccgtgagatcaactagcagaggcttgtgctggagatctgcaaaagacttaaatgccatgaatttatgatacggtttaggagcccaagcatatatttccacagcattctttaaggcaatcaccaaaaatttgatcctttcatatttaacaactttataatgtatacagccttccaagtccccaacagtgatccagccttgtttcttttctacttctgggtcattatgtagtattctgtttcttaaccatgaaagatagtaaactcgtagcttattcttctttcctgaaattgtcacaaggacattcagtccctctagcacatccatctgctgaaatcgcctccggttgatcagattatagactttgccttgcccacttcggtccaaaagcatcaggccattttcagtccccaccagaaggtttacaccccacagagctgcacaaagtatttctgagttgaatcgtttcttgtattttctgatttctggtgtgtcgctatgaggccgaatgttggttgggtttacatttaccaccgaaatctttcttgcttcattgagtttggcctgttcttgcctaagaagttcgctagtaaacagagctgcggctgatgattcctcatcctcttcatcttcatcagtgggagacgtctggtatactctggggtccacaaagggggtgaaggaggctttggtgctgctccccatgccatattcagtcccagagtccatctcctgggaatgggttgagacgcgccccagtccctcagtcggggttccagctggagaatggctctgctgcaccaggtcagggaggttgatgtggccagcaaagccattgctgtcactgtggccagatcgcttcttctctccagacgtctctctaatcatcaaggttccttctcttgaaatactgccgctgaaactgtccgcatgagaggtctccagcccatgcgtccccaccattcccacattgtactgctcgttgctgcctggagctcctgttggtatcagtctgggtatgtcgctgacagccactgtcccatcatgggtctcgctctctccatcttcctcctcttcctcgctactttctgactcctcactggaggaggagtaatcagtcaccttcttcattgggcggtttgtttcttcaatccggagttctcttagttctttggctaatgccgtcagatcctcatctatagcttttttgtagctagctggtcgactgggccgggtaatgtccctggattcttctggtttcaccttcgcaggctcatgggggagcacaggtgatccttctgacttactgttggctcgaactctggtgcgttcactggatcctgcttgtgatccaggctgggagcctccttgggagctgggctgggagctaggggtgctggagctggaggaactgccactgctggtcctctgcaaggggctctccaagatgggctcagttctccggagatcagggttgcttgctctgatgggttgagatcctagtctgggtcccagagcactaccattcccaggagaattctttctggctaatgctggggatatagaagttgttctttgaggcacctttggtggaatgtcttcttcctgtcgtaaccaagagcttcggtcaaacttttcaatgcgagtggggagaggaggattttccgaggtgggatctgagttctggcgtggcatctccacgcggtgggaggtcacgttcagagcctcctgaaacccagagaggccctttgtgggctgctcgtgcactgactgggaggcggtcaaggcaggtccctgggattttacagctaccagatgtgggatctggggatcgactggtctgagcatggggggtgttcgagcaggctgaactccactaatgctgaaggactccgaccttgggggcaggttggggtcagatatcctgttggcaaccttgtgaggcatggcaggggaactttgccggttgagccttgaccgttcttctacctccttggcccatgctggcttctcactaggactcattccttctttgtaatggtacagtggcttcttctccacaggcctctgctcctgccgctgatgctgaagggaaactaagtagtctctttcttgctttagctgcctctgcagtctttctgcttgtctctgttcttccaattgtttgcgcttatattcctgttcatgctccgcacgcctcctctcctcctcccggcgcatctgctcctcatagtgccggcgctgctccctctcctgctgcttccgcagctccttctctcgcctttgttgctcctccagccgccgcctctgctctttctgctcctcgatgcgcttctgacgctcggccagcagctgccgcttgtgctcctcattctcccgctgctgctgctccagctgctgcctccgtagggcctcagaacgctccttgttggccagctgcagcctcagaaagtccctccgcagcgtcgactcccctggcagattcaggatggagctgggctctcctgagtcattctcctcctcttcttcctcacttccactgtactcatactctgtctcatctttttctcctcgcttcttctttgttctatcaatatggtccttgagttgaatgcggacctgtcgctcattaggttggtctcgtataaatggatgcttcatcaattgttctgttgctggtcgctggctgtgattctttaccaagcagctctcaataaatgactggaatttttttgaccacttcttagacttcagccgaggcgctgggttccgggggatgaggaagagagctctcatggggtgcatgtcacagagagggggagcaccttctgccatttcaatggcggtgatacccaaagaccacaagtcactcttgaaatcatatgtggcatctgggttttcatcacaggcaataacttctggtgccatccagtagggagttccaatgaaagtattcctcctgcccactgttcgatcaagctgagcactgactccaaagtccactagtttaacttctgcattttcagtcagcaagacattttgccctttaatatctcgatgaatcactttatgctggtgcaggtgactcagcccccgtaagatttccctgcagatgtatgcaatccactcctctttcaacgtgttaccttttgtgttcttgatcaggtcggtgacagagccagcaccacaaaactccatcaccaaccaaagttggtcatccatgcctggtgggttctttttgataaaagcaccatagtatgtagcaatattccggtgatgagaatatttcttcaacatgttaatttcttgtttgatttcttcctcttcatcccctgtgacatccataaccttgatggctgcaagctggcccgttttgacatgacgacccttataaacttgcccgtatgttccatttccaacaagttccaccaattcaaagatccctgcggggtccctcagagccgagagatctatttcatccaggcttcgagccggggagtcgctcgccatgtctacttcttcgctggagaaatggaccaaaaccaccccgaagcttttcccttggaaattccaccttggtctatttcactcgcgtcctcatgcgggtgtcgcgccagaggccccgggcccagcctcccccgcccaccccagccccacagcgccggatcccgatcctccgcgcgtcggtccgccgggtccgggagcccagcctgcgcggatctccaagccccgagcagcggtgcgtgtgggctgagcgccccgatcggctaagggcgctggggctgcgtgggtgtatttaaatgggacatgcttctttgcttgtgcgtggatggcggctgcattggctgttat

SEQ ID NO: 18404 - RNA, 1220 nt, Homo sapiens
  source 1..1220: mol_type = other RNA
tgactatgatgtgcacctgatcctcgtccttgtccttcttcacatagaacatttttctgaattttttcagctcatggagttcacagaaggtttccagaactaccaacatggcaataaggccaagtagcaggtaacacgtgatcccaatcttatagagctctctgaatttttgattgtagccttccccaggcacataatcccccaggccaatggtgctcagggaaataaaacaaaaataaaaggattccaggaagttccagtcatcctccaggactgagaagacagcggccgggatgaagaagaagcaggacacagtgacaaacccaaggagcacggcatggacgatggccaccacctgcttggagaagccccagcggatgtggaagtagaggaccggcctgcgggtgacgtgcacggtgatgcgctggaccacagccgtcaggaacaggagggtgaagggaatgccaatgacggagtagatgatgcagaaggccttacctccatctgacaagggcacggtgtggccataacctattgcacattcttcaagataccagggcacaaacgggaatgaacattttctgcttttgagctgataaccgttgagcttaaaatcctgtgtatctccagacttgggcatgagtgtggaaatgacttggctaaaagaatcacctgcgcacatgtagattcaacatgggacctacttcttgagttcacagcttctaaataaagtaacaagaaggaaaagaagacttcgcaagtgtgattctgtgcgtagttaaaaaaaattcctatctgatgaggaagaaaacagaaccaaaggtctgcacttctgagcatttctgagttttcatacagtagttctgtcatcccaacttccttgtcaagaacagacttgtaatattgggagccccaggctttctagtcgggtttgggttgtgaaattcttggtgcggccgtccagggccgtctccctcttcccgccgtgccccagaaccaatgagtttccatttatgtccacctaggagctgtccatgacaagctccgcccatggttttccttcatccctgcgactacggagcatcacaccctggcggtcctctggtcagtgcaatctcttcttccgtgcttgtgtttgaatgactgagaaagctaggcactctgttgcctaactccggctttccctgttttaagccaggttgcaggacaggctatttatc

SEQ ID NO: 18405 - RNA, 952 nt, Homo sapiens
  source 1..952: mol_type = other RNA
tgactatgatgtgcacctgatcctcgtccttgtccttcttcacatagaacatttttctgaattttttcagctcatggagttcacagaaggtttccagaactaccaacatggcaataaggccaagtagcaggtaacacgtgatcccaatcttatagagctctctgaatttttgattgtagccttccccaggcacataatcccccaggccaatggtgctcagggaaataaaacaaaaataaaaggattccaggaagttccagtcatcctccaggactgagaagacagcggccgggatgaagaagaagcaggacacagtgacaaacccaaggagcacggcatggacgatggccaccacctgcttggagaagccccagcggatgtggaagtagaggaccggcctgcgggtgacgtgcacggtgatgcgctggaccacagccgtcaggaacaggagggtgaagggaatgccaatgacggagtagatgatgcagaaggccttacctccatctgacaagggcacggtgtggccataacctgtggtggagagcacggtgctggcgaagaagagcgcggaggtgaagtcccagttccagttgcccgaggcgttgctgagcaccgacacgccgtagttgctggcctccagcacccggcccaggaactgctccagctgctgctcagacaggcactcgtgctcctccaagaagcgtcgcttcagcttgcgcagctcctggcgcagcaggtcctcatagggcagctccaccgaggagaagaccactgcgccgaagaccaggtagagcaagtagcccagcaccaggaagccgaagcaccaggccgagcggtgccgctccaccaggcgcacgcacgagctgccggccagggactgcagcatcttctccaccgccgccgccaaggccaacgccgcagaccggccggagcgcggcccgccgcctcttct

SEQ ID NO: 18406 - RNA, 1052 nt, Homo sapiens
  source 1..1052: mol_type = other RNA
tgactgagcttctccccacagcaccaacaatcctgtcagcttcttcccaggcagcagcaggcctcacatccccaccaaaagggacaccattgtgatagcctgggctgcagagatgcacgccctgcagggacagctgtaggtcttggcacagatacagtggcctgggctaatcttgagctgggcctttgcctcctgggttactgatgagaagctctgaggctgaggccagtggatgccccccagacctctccactctccccaagcacccaaggccagttctatgactgtcctggtgagtgccagatgcagggaaagtggccccctgtgtggggcaggtggcttctgcatttctgattagggggccaggaaggaggcattcaggagaaaacaccaagtcagaaaaaaggttcccaggactggggacgaaagactcagaaggaggggaaagaggaagaaagctgtaggggaagggaagggagggggatgagaaaaacgctggggaacaccactgaagttacttcaagctagcaacactggacgctcaggtcttctgttgcatgggttaccgggttacatgccaagggctcagtggctgcctgtggctggtggctcccctgctctgtgctgaggccgctgccgagctgtctattcagagtcagctcctctggtgctggaagatgctggcactcagtgctccatcgcctctcagtgagctggaagttggagtgactcacttgaggcaccagaaatgctcgctgcagtgcagatgttaggacctgggttcagaaagcagatccctaaatgagcctctggggtccacggcttctggtccacgtgcccacggcttggtgaggtctgggaggtctccctgagggaggcaggacttgagtgggaccgtgaagggcagaaataaccacacatacccaggaaaggctcgtgttctgcagtggttaccttacaattcagaatgaactttgaacaaatccctgaagacaacgaggctggccgtggatgtgcagctgccttgcgccttagtgtgtcatctgtaaaat

SEQ ID NO: 18407 - RNA, 472 nt, Homo sapiens
  source 1..472: mol_type = other RNA
tgactgagcttctccccacagtcaccctgatgccccgctcttgctcggctggaggcctcggatctccgtggtgttgagggagccggggcactggagccctggtgacctgcatctcctggcggagccgggaagagctcatggactgtcacagatggacagtgccccgcgggggctggagagcagagtggggctggaaggtggaactcttagccaaagtcttggtttcttttggccagggtcctctttcaatggctggagaaggtggtgctggggggtgaacgctgacctcctcatgtgctgcccctccctcgcctgggcccggtaaagcccccacgtagccccagccagcctggaacatgcttcctgagctcccagctcttggtctttgcacccagtggaggaggaggtcagcccagggagctgagtctgcggtttagggcgtccaggggacgtggaagcatgtgggtcgtct

SEQ ID NO: 18408 - RNA, 3331 nt, Homo sapiens
  source 1..3331: mol_type = other RNA
tgacttctacctcttccaaagactacacagctgcaggcccagcctcagagcagaggtgatatgggtattaccaggctctaatggaaagtgtgctctctcgatatctacttgcagggaagcttctgaaattggtaagggagcacctattgcaaggctcagtgaacaaatggttttggtatttccctttttcatggggcaccagaagggtattttctcctacacaggatcgcatctgaagactttgctgaactgtgttttcctgaagtgaggagatgaaagacctcagataggaaaaacagagagtgagagagagagacagacactgagccaggttcccacacagtttattgagggagccaaagccagtgagaggacgaaggagtcctacttcaacctacttccttaaagctgtgtgcctccagcatgaagggaccttcccagagggcagggcctgccctataaggggccacatgaagccttgtggagactcctgcctctcataccacagcctgtcctaccctaaagacccagacatgacagcagacataatccccaccccaggagggtgctgaggaaacacccttacccatgcccctcccctagagacctcaggaagaaaggccaggacacctgtcctgtgattggccagttgaatcctcaacgtgaagacctggcaggcctggctgacaggtctgttcagatgtggcctcaggcatctactctaggatccaacccctaacattcaaacatgattaaaaacacccaggacacttctcttgctggcagaggccacaccccagataatggcagtcctgccaaactctggccagagatagggacccaagctgactgggtgtgagcacgtaaggagaccactctgccccatggggagaatcttccagggctcagctgaggctcagagcccaggcttatgttattccccatcaaatgccagtgattcctccaaacattccccacaagggagaaagggaggaggaggcagagagcttatcaagaggttcaccctatatggggctggaggttggatctactggggtgaggaaaagggtgtagaggattggggcactggggcaggggcgctggcacattcctcagattctggcatgtcatcctggaagtactcagcctggcggtactgccacagacgcaggttcccgtcccacgaactgctgacaatcttctcttcaaaggggtgccaactgacgtcacgcacacaggccttgtggttggtcagcttcttcacaatgtggccacttagaaggtcgtacacaaccactttgccagtggagcagccactgtagatgaactgctggccagtgctatgaatgggggagaaccggcagcggatgagggtgtgcagcactccgtggccccggtaggtcatcaaggagctgtcccctgggagcttcagcttccgccaggcttttttgggcacttgctgccaccgatagtcccagttttgctgtgtggcagcctggcgtgaagcttccatgccttcccggctggaaaagcgtcggatatcccagagtttgatggtctggtctttagagttggagatcagataccgggcatcacccttgctgtcaatgaaggtgatgccatcctggtgtccagccagtgcacccacaggcttggggtcatcctcccgcatggtgcgtcgatcccacactttgcagatggcatcatctcccccagagaacaggatttgggagcttatatcagcaaaggccactgcattcacatcatcctcatgggactcaatctgaagggtgcgccggttctgttctcggtcaaagacatacaggcagccatcattggcccctcctagtacttctcgtccatctgaggagacagcaatggagaagacagcaaagcgacgctcatctggcctgagatccagggcagtgtgtgtatctccctcaccatagatattgcagatatgaatgtaatcagaccagctagagtagaggaagtggttcccatcaggggtgaaggccacatccaagacgctccagcctacgtcgcgggccttgatgctcttgaatttacggaaacggccatatcggcagtcatagagtcggattgtctggtcttggcaagcagacatgaatatttgaccatctttgctgtagatgccacagaaagccttctgagagtagctatcagtgaagcccagatcattgggcaagaagctggtgcaacattcgaggaaagctgtgcttctgggcggcccgcctaagccccagctgccctgtggccagttccacttgtgtcttgatctcattgaattccagctcccgggtgtcaggggtagcatccacaggtgggttgtatcgatccccaagacgaccatcccaagctctgtcattctcttcctctgagtccaagagggcctgaatgaattgtaaatttgctgcacctcctccctgcaccaacctcacttggcctctgggccagatccacatcttcatcctcttcttcctcttcctcactccgacgcaggccagcccctcttcggggcaagccctcggaggggtctccggacccggatcctgcactgctgctgttccgcgatcccatcttctggtcacagcattcttaggtcctgtgcgggggctcctcctgtcacctccttgggtttggtgaaagcaaagcgtgctctagaaataccagggtctcctgagacggggtagtagctatctctaggagggtgacccttcctcggggctgagatcccttttctttagcctatgccaactaccaaggcgtcgggaacacaaaccttctccaatcctatcgaagtccccggactggggagcgggaggggtgttgggcggtgttggatttccaggtaacctctctgaccgaccaatcgaaatccctctcggaagaaagcgcttcactagcttatctcatctaaccaattagaagccttaggactcaaagaccctcgacgcccccaccttatcgaccaatcagagcgcccccttacaaaggccggcagcagtgacagccaatgaaaatagaatttggcctaacacccctccttcctcgcctcacgcccacgtggtgcgccgggggtgtgtacgccatgagggggaggaagccgagaagcacctcccactgaagccggcggtaaccgccccacgcgagaccacccaccagccaggagcggtcgcaggacccgcagcggcgcgaggccttgtttacaccgactgccgccactgcgttggccaaccgctcctccgtcacgcgcttcgctcgtcacgcatctcgcggcttcctggccggcgggctgcaaacgtcacac

SEQ ID NO: 18409 - RNA, 2889 nt, Homo sapiens
  source 1..2889: mol_type = other RNA
tgacttctacctcttccaaagactacacagctgcaggcccagcctcagagcagaggtgatatgggtattaccaggctctaatggaaagtgtgctctctcgatatctacttgcagggaagcttctgaaattggtaagggagcacctattgcaaggctcagtgaacaaatggttttggtatttccctttttcatggggcaccagaagggtattttctcctacacaggatcgcatctgaagactttgctgaactgtgttttcctgaagtgaggagatgaaagacctcagataggaaaaacagagagtgagagagagagacagacactgagccaggttcccacacagtttattgagggagccaaagccagtgagaggacgaaggagtcctacttcaacctacttccttaaagctgtgtgcctccagcatgaagggaccttcccagagggcagggcctgccctataaggggccacatgaagccttgtggagactcctgcctctcataccacagcctgtcctaccctaaagacccagacatgacagcagacataatccccaccccaggagggtgctgaggaaacacccttacccatgcccctcccctagagacctcaggaagaaaggccaggacacctgtcctgtgattggccagttgaatcctcaacgtgaagacctggcaggcctggctgacaggtctgttcagatgtggcctcaggcatctactctaggatccaacccctaacattcaaacatgattaaaaacacccaggacacttctcttgctggcagaggccacaccccagataatggcagtcctgccaaactctggccagagatagggacccaagctgactgggtgtgagcacgtaaggagaccactctgccccatggggagaatcttccagggctcagctgaggctcagagcccaggcttatgttattccccatcaaatgccagtgattcctccaaacattccccacaagggagaaagggaggaggaggcagagagcttatcaagaggttcaccctatatggggctggaggttggatctactggggtgaggaaaagggtgtagaggattggggcactggggcaggggcgctggcacattcctcagattctggcatgtcatcctggaagtactcagcctggcggtactgccacagacgcaggttcccgtcccacgaactgctgacaatcttctcttcaaaggggtgccaactgacgtcacgcacacaggccttgtggttggtcagcttcttcacaatgtggccacttagaaggtcgtacacaaccactttgccagtggagcagccactgtagatgaactgctggccagtgctatgaatgggggagaaccggcagcggatgagggtgtgcagcactccgtggccccggtaggtcatcaaggagctgtcccctgggagcttcagcttccgccaggcttttttgggcacttgctgccaccgatagtcccagttttgctgtgtggcagcctggcgtgaagcttccatgccttcccggctggaaaagcgtcggatatcccagagtttgatggtctggtctttagagttggagatcagataccgggcatcacccttgctgtcaatgaaggtgatgccatcctggtgtccagccagtgcacccacaggcttggggtcatcctcccgcatggtgcgtcgatcccacactttgcagatggcatcatctcccccagagaacaggatttgggagcttatatcagcaaaggccactgcattcacatcatcctcatgggactcaatctgaagggtgcgccggttctgttctcggtcaaagacatacaggcagccatcattggcccctcctagtacttctcgtccatctgaggagacagcaatggagaagacagcaaagcgacgctcatctggcctgagatccagggcagtgtgtgtatctccctcaccatagatattgcagatatgaatgtaatcagaccagctagagtagaggaagtggttcccatcaggggtgaaggccacatccaagacgctccagcctacgtcgcgggccttgatgctcttgaatttacggaaacggccatatcggcagtcatagagtcggattgtctggtcttggcaagcagacatgaatatttgaccatctttgctgtagatgccacagaaagccttctgagagtagctatcagtgaagcccagatcattgggcaagaagtgagatatcactcgagactgttctccaagggagaagcttccccgatggcagaggccccgttctctctggtgcaacattcgaggaaagctgtgcttctgggcggcccgcctaagccccagctgccctgtggccagttccacttgtgtcttgatctcattgaattccagctcccgggtgtcaggggtagcatccacaggtgggttgtatcgatccccaagacgaccatcccaagctctgtcattctcttcctctgagtccaagagggcctgaatgaattgtaaatttgctgcacctcctccctgcaccaacctcacttggcctctgcggaggagataggccagtacctgggccagatccacatcttcatcctcttcttcctcttcctcactccgacgcaggccagcccctcttcggggcaagccctcggaggggtctccggacccggatcctgcactgctgctgttccgcgatcccatcttctggtcacagcattcttaggtcctgtgcgggggctcctcctgtcacctccagccaggagcggtcgcaggacccgcagcggcgcgaggccttgtttacaccgactgccgccactgcgttggccaaccgctcctccgtcacgcgcttcgctcgtcacgcatctcgcggcttcctggccggcgggctgcaaacgtcacac

SEQ ID NO: 18410 - RNA, 3419 nt, Homo sapiens
  source 1..3419: mol_type = other RNA
tgacttctacctcttccaaagactacacagctgcaggcccagcctcagagcagaggtgatatgggtattaccaggctctaatggaaagtgtgctctctcgatatctacttgcagggaagcttctgaaattggtaagggagcacctattgcaaggctcagtgaacaaatggttttggtatttccctttttcatggggcaccagaagggtattttctcctacacaggatcgcatctgaagactttgctgaactgtgttttcctgaagtgaggagatgaaagacctcagataggaaaaacagagagtgagagagagagacagacactgagccaggttcccacacagtttattgagggagccaaagccagtgagaggacgaaggagtcctacttcaacctacttccttaaagctgtgtgcctccagcatgaagggaccttcccagagggcagggcctgccctataaggggccacatgaagccttgtggagactcctgcctctcataccacagcctgtcctaccctaaagacccagacatgacagcagacataatccccaccccaggagggtgctgaggaaacacccttacccatgcccctcccctagagacctcaggaagaaaggccaggacacctgtcctgtgattggccagttgaatcctcaacgtgaagacctggcaggcctggctgacaggtctgttcagatgtggcctcaggcatctactctaggatccaacccctaacattcaaacatgattaaaaacacccaggacacttctcttgctggcagaggccacaccccagataatggcagtcctgccaaactctggccagagatagggacccaagctgactgggtgtgagcacgtaaggagaccactctgccccatggggagaatcttccagggctcagctgaggctcagagcccaggcttatgttattccccatcaaatgccagtgattcctccaaacattccccacaagggagaaagggaggaggaggcagagagcttatcaagaggttcaccctatatggggctggaggttggatctactggggtgaggaaaagggtgtagaggattggggcactggggcaggggcgctggcacattcctcagattctggcatgtcatcctggaagtactcagcctggcggtactgccacagacgcaggttcccgtcccacgaactgctgacaatcttctcttcaaaggggtgccaactgacgtcacgcacacaggccttgtggttggtcagcttcttcacaatgtggccacttagaaggtcgtacacaaccactttgccagtggagcagccactgtagatgaactgctggccagtgctatgaatgggggagaaccggcagcggatgagggtgtgcagcactccgtggccccggtaggtcatcaaggagctgtcccctgggagcttcagcttccgccaggcttttttgggcacttgctgccaccgatagtcccagttttgctgtgtggcagcctggcgtgaagcttccatgccttcccggctggaaaagcgtcggatatcccagagtttgatggtctggtctttagagttggagatcagataccgggcatcacccttgctgtcaatgaaggtgatgccatcctggtgtccagccagtgcacccacaggcttggggtcatcctcccgcatggtgcgtcgatcccacactttgcagatggcatcatctcccccagagaacaggatttgggagcttatatcagcaaaggccactgcattcacatcatcctcatgggactcaatctgaagggtgcgccggttctgttctcggtcaaagacatacaggcagccatcattggcccctcctagtacttctcgtccatctgaggagacagcaatggagaagacagcaaagcgacgctcatctggcctgagatccagggcagtgtgtgtatctccctcaccatagatattgcagatatgaatgtaatcagaccagctagagtagaggaagtggttcccatcaggggtgaaggccacatccaagacgctccagcctacgtcgcgggccttgatgctcttgaatttacggaaacggccatatcggcagtcatagagtcggattgtctggtcttggcaagcagacatgaatatttgaccatctttgctgtagatgccacagaaagccttctgagagtagctatcagtgaagcccagatcattgggcaagaagtgagatatcactcgagactgttctccaagggagaagcttccccgatggcagaggccccgttctctctggtgcaacattcgaggaaagctgtgcttctgggcggcccgcctaagccccagctgccctgtggccagttccacttgtgtcttgatctcattgaattccagctcccgggtgtcaggggtagcatccacaggtgggttgtatcgatccccaagacgaccatcccaagctctgtcattctcttcctctgagtccaagagggcctgaatgaattgtaaatttgctgcacctcctccctgcaccaacctcacttggcctctgcggaggagataggccagtacctgggccagatccacatcttcatcctcttcttcctcttcctcactccgacgcaggccagcccctcttcggggcaagccctcggaggggtctccggacccggatcctgcactgctgctgttccgcgatcccatcttctggtcacagcattcttaggtcctgtgcgggggctcctcctgtcacctccttgggtttggtgaaagcaaagcgtgctctagaaataccagggtctcctgagacggggtagtagctatctctaggagggtgacccttcctcggggctgagatcccttttctttagcctatgccaactaccaaggcgtcgggaacacaaaccttctccaatcctatcgaagtccccggactggggagcgggaggggtgttgggcggtgttggatttccaggtaacctctctgaccgaccaatcgaaatccctctcggaagaaagcgcttcactagcttatctcatctaaccaattagaagccttaggactcaaagaccctcgacgcccccaccttatcgaccaatcagagcgcccccttacaaaggccggcagcagtgacagccaatgaaaatagaatttggcctaacacccctccttcctcgcctcacgcccacgtggtgcgccgggggtgtgtacgccatgagggggaggaagccgagaagcacctcccactgaagccggcggtaaccgccccacgcgagaccacccaccagccaggagcggtcgcaggacccgcagcggcgcgaggccttgtttacaccgactgccgccactgcgttggccaaccgctcctccgtcacgcgcttcgctcgtcacgcatctcgcggcttcctggccggcgggctgcaaacgtcacac

SEQ ID NO: 18411 - RNA, 2946 nt, Homo sapiens
  source 1..2946: mol_type = other RNA
tgacttctacctcttccaaagactacacagctgcaggcccagcctcagagcagaggtgatatgggtattaccaggctctaatggaaagtgtgctctctcgatatctacttgcagggaagcttctgaaattggtaagggagcacctattgcaaggctcagtgaacaaatggttttggtatttccctttttcatggggcaccagaagggtattttctcctacacaggatcgcatctgaagactttgctgaactgtgttttcctgaagtgaggagatgaaagacctcagataggaaaaacagagagtgagagagagagacagacactgagccaggttcccacacagtttattgagggagccaaagccagtgagaggacgaaggagtcctacttcaacctacttccttaaagctgtgtgcctccagcatgaagggaccttcccagagggcagggcctgccctataaggggccacatgaagccttgtggagactcctgcctctcataccacagcctgtcctaccctaaagacccagacatgacagcagacataatccccaccccaggagggtgctgaggaaacacccttacccatgcccctcccctagagacctcaggaagaaaggccaggacacctgtcctgtgattggccagttgaatcctcaacgtgaagacctggcaggcctggctgacaggtctgttcagatgtggcctcaggcatctactctaggatccaacccctaacattcaaacatgattaaaaacacccaggacacttctcttgctggcagaggccacaccccagataatggcagtcctgccaaactctggccagagatagggacccaagctgactgggtgtgagcacgtaaggagaccactctgccccatggggagaatcttccagggctcagctgaggctcagagcccaggcttatgttattccccatcaaatgccagtgattcctccaaacattccccacaagggagaaagggaggaggaggcagagagcttatcaagaggttcaccctatatggggctggaggttggatctactggggtgaggaaaagggtgtagaggattggggcactggggcaggggcgctggcacattcctcagattctggcatgtcatcctggaagtactcagcctggcggtactgccacagacgcaggttcccgtcccacgaactgctgacaatcttctcttcaaaggggtgccaactgacgtcacgcacacaggccttgtggttggtcagcttcttcacaatgtggccacttagaaggtcgtacacaaccactttgccagtggagcagccactgtagatgaactgctggccagtgctatgaatgggggagaaccggcagcggatgagggtgtgcagcactccgtggccccggtaggtcatcaaggagctgtcccctgggagcttcagcttccgccaggcttttttgggcacttgctgccaccgatagtcccagttttgctgtgtggcagcctggcgtgaagcttccatgccttcccggctggaaaagcgtcggatatcccagagtttgatggtctggtctttagagttggagatcagataccgggcatcacccttgctgtcaatgaaggtgatgccatcctggtgtccagccagtgcacccacaggcttggggtcatcctcccgcatggtgcgtcgatcccacactttgcagatggcatcatctcccccagagaacaggatttgggagcttatatcagcaaaggccactgcattcacatcatcctcatgggactcaatctgaagggtgcgccggttctgttctcggtcaaagacatacaggcagccatcattggcccctcctagtacttctcgtccatctgaggagacagcaatggagaagacagcaaagcgacgctcatctggcctgagatccagggcagtgtgtgtatctccctcaccatagatattgcagatatgaatgtaatcagaccagctagagtagaggaagtggttcccatcaggggtgaaggccacatccaagacgctccagcctacgtcgcgggccttgatgctcttgaatttacggaaacggccatatcggcagtcatagagtcggattgtctggtcttggcaagcagacatgaatatttgaccatctttgctgtagatgccacagaaagccttctgagagtagctatcagtgaagcccagatcattgggcaagaagtgagatatcactcgagactgttctccaagggagaagcttccccgatggcagaggccccgttctctctggtgcaacattcgaggaaagctgtgcttctgggcggcccgcctaagccccagctgccctgtggccagttccacttgtgtcttgatctcattgaattccagctcccgggtgtcaggggtagcatccacaggtgggttgtatcgatccccaagacgaccatcccaagctctgtcattctcttcctctgagtccaagagggcctgcggaggagataggccagtacctgggccagatccacatcttcatcctcttcttcctcttcctcactccgacgcaggccagcccctcttcggggcaagccctcggaggggtctccggacccggatcctgcactgctgctgttccgcgatcccatcttctggtcacagcattcttaggtcctgtgcgggggctcctcctgtcacctccttgggtttggtgaaagcaaagcgtgctctagaaataccagggtctcctgagacggggtagtagctatctctaggagggtgacccttcctcggggctgagatcccttttctttagcctatgccaactaccaaggcgtcgggaacacaaaccttctccaatcctgtgaagcaaagaaagcaagagtgaaccgtagtgcgctaccctagctcaccaactgaagaaagatttgttttctacaccaaactcacctatcgaagtc

SEQ ID NO: 18412 - RNA, 2771 nt, Homo sapiens
  source 1..2771: mol_type = other RNA
tgacttctacctcttccaaagactacacagctgcaggcccagcctcagagcagaggtgatatgggtattaccaggctctaatggaaagtgtgctctctcgatatctacttgcagggaagcttctgaaattggtaagggagcacctattgcaaggctcagtgaacaaatggttttggtatttccctttttcatggggcaccagaagggtattttctcctacacaggatcgcatctgaagactttgctgaactgtgttttcctgaagtgaggagatgaaagacctcagataggaaaaacagagagtgagagagagagacagacactgagccaggttcccacacagtttattgagggagccaaagccagtgagaggacgaaggagtcctacttcaacctacttccttaaagctgtgtgcctccagcatgaagggaccttcccagagggcagggcctgccctataaggggccacatgaagccttgtggagactcctgcctctcataccacagcctgtcctaccctaaagacccagacatgacagcagacataatccccaccccaggagggtgctgaggaaacacccttacccatgcccctcccctagagacctcaggaagaaaggccaggacacctgtcctgtgattggccagttgaatcctcaacgtgaagacctggcaggcctggctgacaggtctgttcagatgtggcctcaggcatctactctaggatccaacccctaacattcaaacatgattaaaaacacccaggacacttctcttgctggcagaggccacaccccagataatggcagtcctgccaaactctggccagagatagggacccaagctgactgggtgtgagcacgtaaggagaccactctgccccatggggagaatcttccagggctcagctgaggctcagagcccaggcttatgttattccccatcaaatgccagtgattcctccaaacattccccacaagggagaaagggaggaggaggcagagagcttatcaagaggttcaccctatatggggctggaggttggatctactggggtgaggaaaagggtgtagaggattggggcactggggcaggggcgctggcacattcctcagattctggcatgtcatcctggaagtactcagcctggcggtactgccacagacgcaggttcccgtcccacgaactgctgacaatcttctcttcaaaggggtgccaactgacgtcacgcacacaggccttgtggttggtcagcttcttcacaatgtggccacttagaaggtcgtacacaaccactttgccagtggagcagccactgtagatgaactgctggccagtgctatgaatgggggagaaccggcagcggatgagggtgtgcagcactccgtggccccggtaggtcatcaaggagctgtcccctgggagcttcagcttccgccaggcttttttgggcacttgctgccaccgatagtcccagttttgctgtgtggcagcctggcgtgaagcttccatgccttcccggctggaaaagcgtcggatatcccagagtttgatggtctggtctttagagttggagatcagataccgggcatcacccttgctgtcaatgaaggtgatgccatcctggtgtccagccagtgcacccacaggcttggggtcatcctcccgcatggtgcgtcgatcccacactttgcagatggcatcatctcccccagagaacaggatttgggagcttatatcagcaaaggccactgcattcacatcatcctcatgggactcaatctgaagggtgcgccggttctgttctcggtcaaagacatacaggcagccatcattggcccctcctagtacttctcgtccatctgaggagacagcaatggagaagacagcaaagcgacgctcatctggcctgagatccagggcagtgtgtgtatctccctcaccatagatattgcagatatgaatgtaatcagaccagctagagtagaggaagtggttcccatcaggggtgaaggccacatccaagacgctccagcctacgtcgcgggccttgatgctcttgaatttacggaaacggccatatcggcagtcatagagtcggattgtctggtcttggcaagcagacatgaatatttgaccatctttgctgtagatgccacagaaagccttctgagagtagctatcagtgaagcccagatcattgggcaagaagtgagatatcactcgagactgttctccaagggagaagcttccccgatggcagaggccccgttctctctggtgcaacattcgaggaaagctgtgcttctgggcggcccgcctaagccccagctgccctgtggccagttccacttgtgtcttgatctcattgaattccagctcccgggtgtcaggggtagcatccacaggtgggttgtatcgatccccaagacgaccatcccaagctctgtcattctcttcctctgagtccaagagggcctgggccagatccacatcttcatcctcttcttcctcttcctcactccgacgcaggccagcccctcttcggggcaagccctcggaggggtctccggacccggatcctgcactgctgctgttccgcgatcccatcttctggtcacagcattcttaggtcctgtgcgggggctcctcctgtcacctccttctccaatcctgtgaagcaaagaaagcaagagtgaaccgtagtgcgctaccctagctcaccaactgaagaaagatttgttttctacaccaaactcacctatcgaag

SEQ ID NO: 18413 - RNA, 495 nt, Homo sapiens
  source 1..495: mol_type = other RNA
tgacttctacctcttccaaagcatcaatcctttccctctgccttctcctaccatcctgaagaggcaataataataacaaggacaaacatttatttggcactgtttctgttttaagcacttgactctatgcttctaaaatcacaggaaatagactatttccgccgaatataaactcattcttgccttcagaacatcttacctgcatgggcagacagggcctccagaggacagctgcattccaaaaaagcctgaaataaagcattaggcaagtatctgcctacagggctgaacacatagtgtttttaacaacattttctgcaagttaggtgagagtttcttggctatagataggatttgaacttaccagcatataatccccagaagagcttggactagtcttttttccatatgacggtagtacttgacacattgaagagacttacttggtgtttgttatgaattaataagcagatgaatgaatgaatcaaaagttga

SEQ ID NO: 18414 - RNA, 50 nt, Homo sapiens
  source 1..50: mol_type = other RNA
tgagacaggcttatgctgctatccttcaaaagaacacatccacccagcta

SEQ ID NO: 18415 - RNA, 2079 nt, Homo sapiens
  source 1..2079: mol_type = other RNA
tgagacctctgggttctgagctgcagggccatcttctgggatcacccgctggaagtgggttcctggaagcatctcatcaaagctggatctggcctcggggtggcgcaacagggatttgggggtgaagataattaacggcttccggaatggcagcaggatctggcgtcgtagcacgtggaagaagttgccaggagtggagcagttgacaacaacccaattgcagtcatatagctgattgatgtcgaagttggcttctttaaggtctggcaggacatctgggtcatcgttgcacatctgcaagaaccgctctgggcgggcggaggaatgttctggacccatgccctccatgccatggggcagcagcaacacgatgccattctgccgcacccacttggcttgtcccgggcagatgaactggtcgatgatacactgggccgtgttgtggaagtcaccaaattgggcttcccagaggaccagggcattaggactggccatggcgaagcccagctcaaagcccagcacgccgtactcagacagtgagctgttgcacacagtatagggggcctgattgggccagagatggttcatggggatgcaggttctcttgtccacattctggtcatggagcacatggtggcggtggctgaatgtgccccgctccacgtcctggccgctcagccgaatgtggatgccctccttcaggagcgagccaaacgccatgtactccgctagagcccagtccacagtccggttcttcaccatttccccacgagtcttcaagatccggctcagccctccatgaatagtaaagttttccacaggcacagaactagccacattcccgatgtgtgtcagaatatcctccgtcagacccgtggaggggcaggacatgctcctgggctgcccgtccagggtgaagaagccaggccagggagagtccagccagtgcttaatgtgcaagatcttctcatctttagatctggcaaaagcttcctcacagatcttatcatacttggaaatttcctcctcatactcaggctggttgaccacaccctgcgacaccagcagctcagcgtacttctgtaacacaggcttctgcttgcggatctgcttgtacatgagcggctgcgtgaacatgggctcatccatctcgttgtggccgttgcgccggtaacacaccaaatcgacaaccacgtccttgtggaaggtgctcctccactcggccgccactttgcacacgtacatgacagcctcggggtcatctgagttcacgtggaaaatgggggcattcaccactcgggccacgtcagtggggtagggggaggagcgggccatccgagggtcggtggtgaagccgatctggttgttgacgaccacgtgcacggtgccatgagttgtgtaggatggcaggtcgctgaggtggaaggtctcgtacacaatgccctggccagcaaatgcagcatccccatgcaacaggatggacatgacctttttcccttcagtgtcgccacagtaaaactgttcggctttggtcttgcccatcaccacggggtcagcggcctcaaggtgggaagggttggccaccaaggacaaggtaatgttcctgtcggtgacacgattgatcctgcggtgatacatgcccaggtggtacttcacatctccggagccctcatcagctgcctccagctttgaatcgaattgacagaagatctgttccagctccttcctgatgacatttgcaagcacgttcagccgccctctgtgtggcatgcccatgatcacgtagtccacgccattctcactagacttgtcaatgatggtcttgagggcagggatcagtacctcgcagccttctagaccaaagcgcttctcagaggaccacttccgctgtaggaactcctcaaacctccagccgacggatgatctcccgcagaggaagtgctgattcctgtcccccgatgaaagtggtggtgggcaagtggaagaccttgtcgaggtcagactcatccaggccatagaacccaagtttgtctgtggatgagataatgtcagcgggcacggaggagtccagatcagcat

SEQ ID NO: 18416 - RNA, 2748 nt, Homo sapiens
  source 1..2748: mol_type = other RNA
tgagacctctgggttctgagctgcagggccatcttctgggatcacccgctggaagtgggttcctggaagcatctcatcaaagctggatctggcctcggggtggcgcaacagggatttgggggtgaagataattaacggcttccggaatggcagcaggatctggcgtcgtagcacgtggaagaagttgccaggagtggagcagttgacaacaacccaattgcagtcatatagctgattgatgtcgaagttggcttctttaaggtctggcaggacatctgggtcatcgttgcacatctgcaagaaccgctctgggcgggcggaggaatgttctggacccatgccctccatgccatggggcagcagcaacacgatgccattctgccgcacccacttggcttgtcccgggcagatgaactggtcgatgatacactgggccgtgttgtggaagtcaccaaattgggcttcccagaggaccagggcattaggactggccatggcgaagcccagctcaaagcccagcacgccgtactcagacagtgagctgttgcacacagtatagggggcctgattgggccagagatggttcatggggatgcaggttctcttgtccacattctggtcatggagcacatggtggcggtggctgaatgtgccccgctccacgtcctggccgctcagccgaatgtggatgccctccttcaggagcgagccaaacgccatgtactccgctagagcccagtccacagtccggttcttcaccatttccccacgagtcttcaagatccggctcagccctccatgaatagtaaagttttccacaggcacagaactagccacattcccgatgtgtgtcagaatatcctccgtcagacccgtggaggggcaggacatgctcctgggctgcccgtccagggtgaagaagccaggccagggagagtccagccagtgcttaatgtgcaagatcttctcatctttagatctggcaaaagcttcctcacagatcttatcatacttggaaatttcctcctcatactcaggctggttgaccacaccctgcgacaccagcagctcagcgtacttctgtaacacaggcttctgcttgcggatctgcttgtacatgagcggctgcgtgaacatgggctcatccatctcgttgtggccgttgcgccggtaacacaccaaatcgacaaccacgtccttgtggaaggtgctcctccactcggccgccactttgcacacgtacatgacagcctcggggtcatctgagttcacgtggaaaatgggggcattcaccactcgggccacgtcagtggggtagggggaggagcgggccatccgagggtcggtggtgaagccgatctggttgttgacgaccacgtgcacggtgccatgagttgtgtaggatggcaggtcgctgaggtggaaggtctcgtacacaatgccctggccagcaaatgcagcatccccatgcaacaggatggacatgacctttttcccttcagtgtcgccacagtaaaactgttcggctttggtcttgcccatcaccacggggtcagcggcctcaaggtgggaagggttggccaccaaggacaaggtaatgttcctgtcggtgacacgattgatcctgcggtgatacatgcccaggtggtacttcacatctccggagccctcatcagctgcctccagctttgaatcgaattgacagaagatctgttccagctccttcctgatgacatttgcaagcacgttcagccgccctctgtgtggcatgcccatgatcacgtagtccacgccattctcactagacttgtcaatgatggtcttgagggcagggatcagtacctcgcagccttctagaccaaagcgcttctcagaggaccacttccgctgtaggaactcctcaaacctggtggaccgcacaagcctggccagcagggtccgtttctcctcatttgtgaactgcatgatcccaggggtctcaaacttctgccggatccactggcactgctccaggtcattgatgaacatgaactccaccccaatatgctggcagtaggccatctccagccgacggatgatctcccgcagaggaagtgctgattcctgtcccccgatgaaagtggtggtgggcaagtggaagaccttgtcgaggtcagactcatccaggccatagaacccaagtttgtctgtggatgagataatgtcagcgggcacggaggagtccagatcagcatccaaaatccccagggggtccagctgtgctacatggtgccctcgtatctgatatgccctgatgagcgactgcactgccaggtggtcctccacgagcttgtccacgttgggctgtgcttctaccagggactgtgcatgggccacagcagccagggagcctcggctcaggggaaggggactctggtaggcagtgcccggtggggctccggcattcgtgttgcgaaaaaaaatgtcccatgacttatgtacacttttggggttttccagccaagcacagtacatctcctccacatagttcgaactagtcccactgagaaagggctcagcagcaacaggtgcagaatagcaccgaatctgttgaaatgtcctagctgctgctggtctgttttgtgaaaatgtcttaacagtctgggaagccgtcaatggcctcaacttagcagcacaagtccttaaatgaaacatttttgtcctgaagtttttcacaactgcctgtctccggctcagctccacccgaat

SEQ ID NO: 18417 - RNA, 2736 nt, Homo sapiens
  source 1..2736: mol_type = other RNA
tgagacctctgggttctgagctgcagggccatcttctgggatcacccgctggaagtgggttcctggaagcatctcatcaaagctggatctggcctcggggtggcgcaacagggatttgggggtgaagataattaacggcttccggaatggcagcaggatctggcgtcgtagcacgtggaagaagttgccaggagtggagcagttgacaacaacccaattgcagtcatatagctgattgatgtcgaagttggcttctttaaggtctggcaggacatctgggtcatcgttgcacatctgcaagaaccgctctgggcgggcggaggaatgttctggacccatgccctccatgccatggggcagcagcaacacgatgccattctgccgcacccacttggcttgtcccgggcagatgaactggtcgatgatacactgggccgtgttgtggaagtcaccaaattgggcttcccagaggaccagggcattaggactggccatggcgaagcccagctcaaagcccagcacgccgtactcagacagtgagctgttgcacacagtatagggggcctgattgggccagagatggttcatggggatgcaggttctcttgtccacattctggtcatggagcacatggtggcggtggctgaatgtgccccgctccacgtcctggccgctcagccgaatgtggatgccctccttcaggagcgagccaaacgccatgtactccgctagagcccagtccacagtccggttcttcaccatttccccacgagtcttcaagatccggctcagccctccatgaatagtaaagttttccacaggcacagaactagccacattcccgatgtgtgtcagaatatcctccgtcagacccgtggaggggcaggacatgctcctgggctgcccgtccagggtgaagaagccaggccagggagagtccagccagtgcttaatgtgcaagatcttctcatctttagatctggcaaaagcttcctcacagatcttatcatacttggaaatttcctcctcatactcaggctggttgaccacaccctgcgacaccagcagctcagcgtacttctgtaacacaggcttctgcttgcggatctgcttgtacatgagcggctgcgtgaacatgggctcatccatctcgttgtggccgttgcgccggtaacacaccaaatcgacaaccacgtccttgtggaaggtgctcctccactcggccgccactttgcacacgtacatgacagcctcggggtcatctgagttcacgtggaaaatgggggcattcaccactcgggccacgtcagtggggtagggggaggagcgggccatccgagggtcggtggtgaagccgatctggttgttgacgaccacgtgcacggtgccatgagttgtgtaggatggcaggtcgctgaggtggaaggtctcgtacacaatgccctggccagcaaatgcagcatccccatgcaacaggatggacatgacctttttcccttcagtgtcgccacagtaaaactgttcggctttggtcttgcccatcaccacggggtcagcggcctcaaggtgggaagggttggccaccaaggacaaggtaatgttcctgtcggtgacacgattgatcctgcggtgatacatgcccaggtggtacttcacatctccggagccctcatcagctgcctccagctttgaatcgaattgacagaagatctgttccagctccttcctgatgacatttgcaagcacgttcagccgccctctgtgtggcatgcccatgatcacgtagtccacgccattctcactagacttgtcaatgatggtcttgagggcagggatcagtacctcgcagccttctagaccaaagcgcttctcagaggaccacttccgctgtaggaactcctcaaacctggtggaccgcacaagcctggccagcagggtccgtttctcctcatttgtgaactgcatgatcccaggggtctcaaacttctgccggatccactggcactgctccaggtcattgatgaacatgaactccaccccaatatgctggcagtaggccatctccagccgacggatgatctcccgcagaggaagtgctgattcctgtcccccgatgaaagtggtggtgggcaagtggaagaccttgtcgaggtcagactcatccaggccatagaaccccacgtttgaagaaacagttactggagcatcatcaaaatttacacaactaattccgagaggatcaagttttgcaatgtggtgacccctgacctgatatgccctgatgagcgactgcactgccaggtggtcctccacgagcttgtccacgttgggctgtgcttctaccagggactgtgcatgggccacagcagccagggagcctcggctcaggggaaggggactctggtaggcagtgcccggtggggctccggcattcgtgttgcgaaaaaaaatgtcccatgacttatgtacacttttggggttttccagccaagcacagtacatctcctccacatagttcgaactagtcccactgagaaagggctcagcagcaacaggtgcagaatagcaccgaatctgttgaaatgtcctagctgctgctggtctgttttgtgaaaatgtcttaacagtctgggaagccgtcaatggcctcaacttagcagcacaagtccttaaatgaaacatttttgtcctgaagtttttcacaactgcctgtctccggctcagctccacccgaat

SEQ ID NO: 18418 - RNA, 2917 nt, Homo sapiens
  source 1..2917: mol_type = other RNA
tgagacctctgggttctgagctgcagggccatcttctgggatcacccgctggaagtgggttcctggaagcatctcatcaaagctggatctggcctcggggtggcgcaacagggatttgggggtgaagataattaacggcttccggaatggcagcaggatctggcgtcgtagcacgtggaagaagttgccaggagtggagcagttgacaacaacccaattgcagtcatatagctgattgatgtcgaagttggcttctttaaggtctggcaggacatctgggtcatcgttgcacatctgcaagaaccgctctgggcgggcggaggaatgttctggacccatgccctccatgccatggggcagcagcaacacgatgccattctgccgcacccacttggcttgtcccgggcagatgaactggtcgatgatacactgggccgtgttgtggaagtcaccaaattgggcttcccagaggaccagggcattaggactggccatggcgaagcccagctcaaagcccagcacgccgtactcagacagtgagctgttgcacacagtatagggggcctgattgggccagagatggttcatggggatgcaggttctcttgtccacattctggtcatggagcacatggtggcggtggctgaatgtgccccgctccacgtcctggccgctcagccgaatgtggatgccctccttcaggagcgagccaaacgccatgtactccgctagagcccagtccacagtccggttcttcaccatttccccacgagtcttcaagatccggctcagccctccatgaatagtaaagttttccacaggcacagaactagccacattcccgatgtgtgtcagaatatcctccgtcagacccgtggaggggcaggacatgctcctgggctgcccgtccagggtgaagaagccaggccagggagagtccagccagtgcttaatgtgcaagatcttctcatctttagatctggcaaaagcttcctcacagatcttatcatacttggaaatttcctcctcatactcaggctggttgaccacaccctgcgacaccagcagctcagcgtacttctgtaacacaggcttctgcttgcggatctgcttgtacatgagcggctgcgtgaacatgggctcatccatctcgttgtggccgttgcgccggtaacacaccaaatcgacaaccacgtccttgtggaaggtgctcctccactcggccgccactttgcacacgtacatgacagcctcggggtcatctgagttcacgtggaaaatgggggcattcaccactcgggccacgtcagtggggtagggggaggagcgggccatccgagggtcggtggtgaagccgatctggttgttgacgaccacgtgcacggtgccatgagttgtgtaggatggcaggtcgctgaggtggaaggtctcgtacacaatgccctggccagcaaatgcagcatccccatgcaacaggatggacatgacctttttcccttcagtgtcgccacagtaaaactgttcggctttggtcttgcccatcaccacggggtcagcggcctcaaggtgggaagggttggccaccaaggacaaggtaatgttcctgtcggtgacacgattgatcctgcggtgatacatgcccaggtggtacttcacatctccggagccctcatcagctgcctccagctttgaatcgaattgacagaagatctgttccagctccttcctgatgacatttgcaagcacgttcagccgccctctgtgtggcatgcccatgatcacgtagtccacgccattctcactagacttgtcaatgatggtcttgagggcagggatcagtacctcgcagccttctagaccaaagcgcttctcagaggaccacttccgctgtaggaactcctcaaacctggtggaccgcacaagcctggccagcagggtccgtttctcctcatttgtgaactgcatgatcccaggggtctcaaacttctgccggatccactggcactgctccaggtcattgatgaacatgaactccaccccaatatgctggcagtaggccatctccagccgacggatgatctcccgcagaggaagtgctgattcctgtcccccgatgaaagtggtggtgggcaagtggaagaccttgtcgaggtcagactcatccaggccatagaaccctcctactgttagcattcgaagtcgttccttgaaaactgcaagatcaagtttgtctgtggatgagataatgtcagcgggcacggaggagtccagatcagcatccaaaatccccagggggtccagctgtgctacatggtgccctcgtatctgatatgccctgatgagcgactgcactgccaggtggtcctccacgagcttgtccacgttgggctgtgcttctaccagggactgtgcatgggccacagcagccagggagcctcggctcaggggaaggggactctggtaggcagtgcccggtggggctccggcattcgtgttgcgaaaaaaaatgtcccatgacttatgtacacttttggggttttccagccaagcacagtacatctcctccacatagttcgaactagtcccactgagaaagggctcagcagcaacaggtgcagaatagcaccgaatctgttgaaatgtcctagctgctgctggtctgttttgtgaaaatgtcttaacagtctgggaagccgtcaatggcctcaacttagcagcacaagtccttaaatgaaacatttttgtcctgaagtttttcacaactgccgagtggggaaacccagccaggcctgtttgttcagattcttcttggcctctctgtgcaggattccttcctgtgggtgtgaggcaggactcctgaagtgggtgtcttgtgacctgtctccggctcagctccacccgaatgaggcgccgacac

SEQ ID NO: 18419 - RNA, 2848 nt, Homo sapiens
  source 1..2848: mol_type = other RNA
tgagacctctgggttctgagctgcagggccatcttctgggatcacccgctggaagtgggttcctggaagcatctcatcaaagctggatctggcctcggggtggcgcaacagggatttgggggtgaagataattaacggcttccggaatggcagcaggatctggcgtcgtagcacgtggaagaagttgccaggagtggagcagttgacaacaacccaattgcagtcatatagctgattgatgtcgaagttggcttctttaaggtctggcaggacatctgggtcatcgttgcacatctgcaagaaccgctctgggcgggcggaggaatgttctggacccatgccctccatgccatggggcagcagcaacacgatgccattctgccgcacccacttggcttgtcccgggcagatgaactggtcgatgatacactgggccgtgttgtggaagtcaccaaattgggcttcccagaggaccagggcattaggactggccatggcgaagcccagctcaaagcccagcacgccgtactcagacagtgagctgttgcacacagtatagggggcctgattgggccagagatggttcatggggatgcaggttctcttgtccacattctggtcatggagcacatggtggcggtggctgaatgtgccccgctccacgtcctggccgctcagccgaatgtggatgccctccttcaggagcgagccaaacgccatgtactccgctagagcccagtccacagtccggttcttcaccatttccccacgagtcttcaagatccggctcagccctccatgaatagtaaagttttccacaggcacagaactagccacattcccgatgtgtgtcagaatatcctccgtcagacccgtggaggggcaggacatgctcctgggctgcccgtccagggtgaagaagccaggccagggagagtccagccagtgcttaatgtgcaagatcttctcatctttagatctggcaaaagcttcctcacagatcttatcatacttggaaatttcctcctcatactcaggctggttgaccacaccctgcgacaccagcagctcagcgtacttctgtaacacaggcttctgcttgcggatctgcttgtacatgagcggctgcgtgaacatgggctcatccatctcgttgtggccgttgcgccggtaacacaccaaatcgacaaccacgtccttgtggaaggtgctcctccactcggccgccactttgcacacgtacatgacagcctcggggtcatctgagttcacgtggaaaatgggggcattcaccactcgggccacgtcagtggggtagggggaggagcgggccatccgagggtcggtggtgaagccgatctggttgttgacgaccacgtgcacggtgccatgagttgtgtaggatggcaggtcgctgaggtggaaggtctcgtacacaatgccctggccagcaaatgcagcatccccatgcaacaggatggacatgacctttttcccttcagtgtcgccacagtaaaactgttcggctttggtcttgcccatcaccacggggtcagcggcctcaaggtgggaagggttggccaccaaggacaaggtaatgttcctgtcggtgacacgattgatcctgcggtgatacatgcccaggtggtacttcacatctccggagccctcatcagctgcctccagctttgaatcgaattgacagaagatctgttccagctccttcctgatgacatttgcaagcacgttcagccgccctctgtgtggcatgcccatgatcacgtagtccacgccattctcactagacttgtcaatgatggtcttgagggcagggatcagtacctcgcagccttctagaccaaagcgcttctcagaggaccacttccgctgtaggaactcctcaaacctggtggaccgcacaagcctggccagcagggtccgtttctcctcatttgtgaactgcatgatcccaggggtctcaaacttctgccggatccactggcactgctccaggtcattgatgaacatgaactccaccccaatatgctggcagtaggccatctccagccgacggatgatctcccgcagaggaagtgctgattcctgtcccccgatgaaagtggtggtgggcaagtggaagaccttgtcgaggtcagactcatccaggccatagaaccctcctactgttagcattcgaagtcgttccttgaaaactgcaagatcaagtttgtctgtggatgagataatgtcagcgggcacggaggagtccagatcagcatccaaaatccccagggggtccagctgtgctacatggtgccctcgtatctgatatgccctgatgagcgactgcactgccaggtggtcctccacgagcttgtccacgttgggctgtgcttctaccagggactgtgcatgggccacagcagccagggagcctcggctcaggggaaggggactctggtaggcagtgcccggtggggctccggcattcgtgttgcgaaaaaaaatgtcccatgacttatgtacacttttggggttttccagccaagcacagtacatctcctccacatagttcgaactagtcccactgagaaagggctcagcagcaacaggtgcagaatagcaccgaatctgttgaaatgtcctagctgctgctggtctgttttgtgaaaatgtcttaacagtctgggaagccgtcaatggcctcaacttagcagcacaagtccttaaatgaaacatttttgtcctgaagtttttcacaactgcctgtctccggctcagctccacccgaatgaggcgccgacaccccactccggggctccaaactctcggccccgccccggcgtat

SEQ ID NO: 18420 - RNA, 2781 nt, Homo sapiens
  source 1..2781: mol_type = other RNA
tgagacctctgggttctgagctgcagggccatcttctgggatcacccgctggaagtgggttcctggaagcatctcatcaaagctggatctggcctcggggtggcgcaacagggatttgggggtgaagataattaacggcttccggaatggcagcaggatctggcgtcgtagcacgtggaagaagttgccaggagtggagcagttgacaacaacccaattgcagtcatatagctgattgatgtcgaagttggcttctttaaggtctggcaggacatctgggtcatcgttgcacatctgcaagaaccgctctgggcgggcggaggaatgttctggacccatgccctccatgccatggggcagcagcaacacgatgccattctgccgcacccacttggcttgtcccgggcagatgaactggtcgatgatacactgggccgtgttgtggaagtcaccaaattgggcttcccagaggaccagggcattaggactggccatggcgaagcccagctcaaagcccagcacgccgtactcagacagtgagctgttgcacacagtatagggggcctgattgggccagagatggttcatggggatgcaggttctcttgtccacattctggtcatggagcacatggtggcggtggctgaatgtgccccgctccacgtcctggccgctcagccgaatgtggatgccctccttcaggagcgagccaaacgccatgtactccgctagagcccagtccacagtccggttcttcaccatttccccacgagtcttcaagatccggctcagccctccatgaatagtaaagttttccacaggcacagaactagccacattcccgatgtgtgtcagaatatcctccgtcagacccgtggaggggcaggacatgctcctgggctgcccgtccagggtgaagaagccaggccagggagagtccagccagtgcttaatgtgcaagatcttctcatctttagatctggcaaaagcttcctcacagatcttatcatacttggaaatttcctcctcatactcaggctggttgaccacaccctgcgacaccagcagctcagcgtacttctgtaacacaggcttctgcttgcggatctgcttgtacatgagcggctgcgtgaacatgggctcatccatctcgttgtggccgttgcgccggtaacacaccaaatcgacaaccacgtccttgtggaaggtgctcctccactcggccgccactttgcacacgtacatgacagcctcggggtcatctgagttcacgtggaaaatgggggcattcaccactcgggccacgtcagtggggtagggggaggagcgggccatccgagggtcggtggtgaagccgatctggttgttgacgaccacgtgcacggtgccatgagttgtgtaggatggcaggtcgctgaggtggaaggtctcgtacacaatgccctggccagcaaatgcagcatccccatgcaacaggatggacatgacctttttcccttcagtgtcgccacagtaaaactgttcggctttggtcttgcccatcaccacggggtcagcggcctcaaggtgggaagggttggccaccaaggacaaggtaatgttcctgtcggtgacacgattgatcctgcggtgatacatgcccaggtggtacttcacatctccggagccctcatcagctgcctccagctttgaatcgaattgacagaagatctgttccagctccttcctgatgacatttgcaagcacgttcagccgccctctgtgtggcatgcccatgatcacgtagtccacgccattctcactagacttgtcaatgatggtcttgagggcagggatcagtacctcgcagccttctagaccaaagcgcttctcagaggaccacttccgctgtaggaactcctcaaacctggtggaccgcacaagcctggccagcagggtccgtttctcctcatttgtgaactgcatgatcccaggggtctcaaacttctgccggatccactggcactgctccaggtcattgatgaacatgaactccaccccaatatgctggcagtaggccatctccagccgacggatgatctcccgcagaggaagtgctgattcctgtcccccgatgaaagtggtggtgggcaagtggaagaccttgtcgaggtcagactcatccaggccatagaaccctcctactgttagcattcgaagtcgttccttgaaaactgcaagatccacgtttgaagaaacagttactggagcatcatcaaaatttacacaactaattccgagaggatcaagttttgcaatgtggtgacccctgacctgatatgccctgatgagcgactgcactgccaggtggtcctccacgagcttgtccacgttgggctgtgcttctaccagggactgtgcatgggccacagcagccagggagcctcggctcaggggaaggggactctggtaggcagtgcccggtggggctccggcattcgtgttgcgaaaaaaaatgtcccatgacttatgtacacttttggggttttccagccaagcacagtacatctcctccacatagttcgaactagtcccactgagaaagggctcagcagcaacaggtgcagaatagcaccgaatctgttgaaatgtcctagctgctgctggtctgttttgtgaaaatgtcttaacagtctgggaagccgtcaatggcctcaacttagcagcacaagtccttaaatgaaacatttttgtcctgaagtttttcacaactgcctgtctccggctcagctccacccgaat

SEQ ID NO: 18421 - RNA, 348 nt, Homo sapiens
  source 1..348: mol_type = other RNA
tgagacctctgggttctgagctttaaatatgggtagttgttctttagaaaatcaaaggtaagaagttacaggtttctttggataacttgccaagacaggcgaaaaccatttccataaatacataaaactgaaggggaagcgcggtcgacttccacagctggtacacagctccgccaggaccttcccagggccctcagcacaccccacgtgcttcacaccagcagaccaggcagtgaccaggaaccagtctcggagagcctcctggcacgacagaaccaccccagcaatggcaactcgaacctgcctgtgaccctccggagtttgttatcatgcctgccactcgcgaga

SEQ ID NO: 18422 - RNA, 366 nt, Homo sapiens
  source 1..366: mol_type = other RNA
tgagacctctgggttctgagctttaaatatgggtagttgttctttagaaaatcgaaggtaagaacttacaggtttctttggacaacttgccaagacagatgaaaaccacctcggtaaatacacaaaactgaagggggagcgcagtcgacttccacagccggtgcacagctctgctccagaccttcccagggcactcagcacgccccacatgcttcggagaaacgccatcgctccggtggatgaggcagtgacccgaccccaatctcggagagcctcctggcaatacacaactccagcaatcacaactggaacccgcgtgcgaccctccggcgtgtgttatcatgcccgccactagcgaggcactat

SEQ ID NO: 18423 - RNA, 367 nt, Homo sapiens
  source 1..367: mol_type = other RNA
tgagacctctgggttctgagctttaaatatgggtagttgttctttagaaaatcgaaggtaagaacttacaggtttctttggacaacttgccaagacagatgaaaaccacctcggtaaatacacaaaactgaagggggagcgcagtcgacttccacagccggtgcacagctctgctccagaccttcccagggcactcagcacgccccacatgcttcggagaaacgccatcgctccggtggatgaggcagtgacccgaccccaatctcggagagcctcctggcaatacacaactccagcaatcacaactggaacccgcgtgcgaccctccggcgtgtgttatcatgcccgccactagcgaggcactatg

SEQ ID NO: 18424 - RNA, 4407 nt, Homo sapiens
  source 1..4407: mol_type = other RNA
tgagagtggaattcacagtatttaaggaatcaatccttgctgcttctgtttatgaagccgagcttcagttttcttgctctgacaatggacacagtgattacctcaagggttgctgtaggagttagatgagatatctataatgtaggaaaggtgtttactacaatgtaactcatggataggggcctatattggttttccattgctgtgtaacaaatttccataaacttagtggcttaaaacaacagacatttattatctttcatttctgtcagaggtccaggcaactgagtggttgatatctctgttcagggtctcacgaggctgaaatcaaggtgtcagttagctgcattcccctctagagacttgactagggaaggattcttttccaaattccttcaagttgttggtagaagtgtttcttgctagcttcaattagggatggatctcagcaactagtgaccactctcaagtctttattatatggccccttttatactcaaaaccagcaacagagaattccccctcacatcaaatccctctcacactttcaatctctatgactcagaaacgggctcacctggctaggtcagacccaccagaatattctccattttggctagctcacagtcgcctgatgagcaatgtaatcatagcagtggtatcatacacacaggtctgcctgcactcaaaggagagtgattatcaaggaatgcacaccaggggcggcaggaatctggcagctatcttagaattctgcctgccaccatttccattaagtgattgttgttgtttgttactgaggcatagatgaagtagcacttatgcaggaaaaaaaccactagtcaatcagaatttcaagttgtatgatgaggtattccatagaaattaaacatgcgtataacagattctcataggtcaggacacatgaaaaatttaaggaaaggatgaggactccttaatttagagggacttctgaaaggtgacttaatgatgacccaacactatatgtgaaatcatgtttggcttcaaaagcactgtgggcagaaaaggagaaaacgtttaatctagagtacacagttatggcattatctggagggaaggataaagctacaaagattgttaaaactaaaatttgttgccaagggagccattcgagctctgtctggagatcttctaaatgagagtaaattattctgtacttgaggtggtttgggcactgtcctccctgaagccaatgtagagataaagtgttgttttcactccttctagtcctgtgattctgcgtctaaggaggcaaaccacctattgaatcagtgctcaccacaggctccattgcagcattgaactgtgtctgtgagaaagaataaggttaagtcaggattccttgattaagacgagttaatataaacactgaaaatccagtgtgctgccagcatagcttttggcagcatcaacacagagaagaaagagctgtaacagaataacagcaaaataacttcgggtccttccttctcctccacccacaaaatcccatttggtgatatgagaatctaaattgctcagtgcttggatgtttggctgtcacatgtcattgttgtgttgaaccttcccaggcatgtacagagctcactgctcaggagattaatgttcaaaagccaaaatgcttgaccaaacttgaaatctatttgtggaatttactgtttcatcattgaaccatgaaaaaataaattcagcaaatatagtcctaatactccagctcatcatgaaatgtctcttaatttcttgacgtgtccatgagttagagacagctgagaaaggtttcattatctttgtctacttacatacattctttctcatttctttttctttttaaaatctaaggctttttttacttgagaaaggagttgttccgattactgtcagtttctctggctgatgtgattttctcatcagaagccttgaacccttctccttttaacttgatagcaaagagaaatcatgatagcttcttttgacatcactttacacaaaaacaaacaaaacaaaacaaaattatcataaactggtagaacaagaagacagcatgtagggaacaaaacaaccatgttcttgattctaatgaggtacatgatttactcctaccatggaaaattcaaatatctacccttgaacttcaacaagcatttatgacttgttgatctacttatagaactaaatgattattttgcaaaacatcatctctgtctttaagtactccctacagaagaaagaaatggaacattagtgtaaacatgatggtcactaagaacttgtggacactgaagaaaggctatggataaatgatccaacaataagagaaagcttctgagtatgcctcagaccagtgactgactgggttttctgggaatatattttttggacaatgggtccaggaagacaataataaatattggaaaaacttcctacagtctataaaatcccttttatttagataatctcactgggaggaaggtaaggagagggatatttattgagagtccgtgacagagagatacactgtgaggtacctttcaggttccatctcattaatttcttaaattgactctaaagaggaatgttacctcaattttatagatgatctccaaaatcctcaaagcttttaagtaacttgtcactctgcataagaatttgcctccaaacttagggattttaaagaactttgtttttcttttttctatgtcacccagagtatttggtcaggaaaagaacttgcagttctcactcatagtcaatttgttggtagtagccactgggtcttcagtccttggaagtctagactgggctggactttcaagatggttcacttaatgactggcagatgtgactggctgtcaactgggacctctcaggggactgttgaccagaatacctacatgtagcctctatagcatggtggtcttaagatagccctacttcttatatgatggacagcctctccagataaagtgttgcacaagatcaagtagaaatgacctgacccttctgagcagcatcaggaattacacagcatcgcttcctccatactctatcggttgaagtaattagaagcccaccaagacttcagggaaagggacataaaagctatcttttgatgaaaggaatgtcaaaatattttggggccatgttttaaaattaccatacttgctcaaaatacaacagcaagtaagtgtccactaaaataaaatacaactcataatgtgtgatggacttttttaaaatttgtaaatggtggaaattgacatcagtgagattaaggctagaagaacgtatacgtttgtaaatcaaatcacaggaaagggaagatgaatatggctttagtcacgtgtggttctaggcaccactgcagaagctttttccatcaactgcatttgattcgctctgtatgttggctgcattttatctattgtagaccactattttcataatgctccagcaacagcaaatgtcatctaaaggaaggaactcctgctccttggttcaaatttgacatactgcagagaacaattttgatacctagtttttgtcacatacaatcacctgttcagtccttatagcagatcctatttgagtcacgtggttagaacaatcctcggtattatagaagattccaaggtgaaaggaatagaaggaaaaatgggtaaaatatggccactctatagaaatcaagagaatttacagtgaatagtgaactaactaccatctctttttgctaagaaacgctttgggacaattttgtaaattttacaaaggaaggaattagtctttatctctcagcaaaccttttgttgaccagaggatccttggaaaaccaaatgaggggctatgtgatttatctgataatgagctagaaatcagagcatatacacacatcttcatttatgtaccacttttcaagtatattcacatgattatttcatttacacacaatagctaagtgttataggacaagttttatcttcattttatagctaagaaatctgagacccagaaagtttaagtgacttaatcccagttacatagggaataaatagcagagctaggacttcaactcagattcctcctcttagaccagtatacttttcaccgcgccacaggttcgcctaatgtaaaacttaagtttcattgatgacatgatacatgggtaaaggttttctctactggaggttccaaccacttgactatctcatcttagagtagctgcctgacaaagcattttggcttctatagagtaaattaaacatgcccttttatgaatgaaattcataaaagtaaatttcctttgccaagattatccttcttaaacatgacatccccttccgtagacaccacttatggtctcccattaca

SEQ ID NO: 18425 - RNA, 168 nt, Homo sapiens
  source 1..168: mol_type = other RNA
tgagcaccacacaggccgggcgcgccatccggtgcagctgggagctgggccatgtgtcctaggccgcggcggggaaggggcgagacccccgcgacctccggcgttccctccctgcccccatctttgggtctttctctgaatggcgcgactccatcagtcctggactct

SEQ ID NO: 18426 - RNA, 177 nt, Homo sapiens
  source 1..177: mol_type = other RNA
tgagcaccacacaggccgggcgcgccatccggtgcagctgggagctgggccatgtgtcctaggccgcggcggggaaggggcgagacccccgcgacctccggcgttccctccctgcccccatctttgggtctttctctgaatggcgcgactccatcagtcctggactctgggcctgag

SEQ ID NO: 18427 - RNA, 1646 nt, Homo sapiens
  source 1..1646: mol_type = other RNA
tgagcaccacacaggccgggcgctcgctcagctgagttgccccaagagttgtgttctgcttgttgtagccagcaaagtgaaggatgctctcagtggccatggccagccccgtgtgctgggacagtcccgatacccagttctgatgtttgttcagatattcctgcaggtgggacttggtgacggtaggtgcccacttcatggcctcctggaggatcatcccacagcgtgcagcgaagtccttcacaatgctctcacgggcttcgtacgtgtcaggaaccgtgatccggtagggggcgtcggggatgtcatagtaaggctgatccttgtgaatatcagcgctcagtgacagtgacagggtctgcaggatgtccagcatggtcttcagcacagtcccgctccagagcaagtggggaaacttatccaccagaccagatagatacttgtctgccaccctccttatcctcttgtggatgtggttgaagttcaccaacaggaactgagcgtgccgctccagctcctcctcgttctccttggtcttggctttatccgccatcatgttcaggaaggcatcgaatactttgtccgcgactgcaatcacacactgcatcatcccagatttgtctttctgaatagctttatcctcaaagtagcagaacattacctggaagcgatcaggatctgttgaacgcagtaccctcatgtactccagccggtacacagagaggaggtaggtggacatggcgaagtccagcttgttgatgagtgcggacacctcgggaggggggtccagcaggttgatgatagtgctgcggagctcactcagctcagcgggggtgaccgtgtcattcttcatggctgagttatactggaggacggaccgcagtggctccttgctgggaaaggtgagcaagggggacttagtggctatttcacagaccccctcgtaccattcttctggccagagtcctgagccctccacagcgaatcccatcagaacggaatacagccagaagtctcggaagagcttctgtaaccgaggcttagcttctttgatgggtggcagtcgtcgggtgagcacagctattacaggaatgagtactcccaagttccctgcactgctagaagcctttagggcagggcccttctcgcttgccctctcgctggctcgcttcccctccagccccagctgcacaaacaactccaacaggttcatgagcagctcatccaccaggtgctcgtcttggatgttggccgcgatgttggccagggcattaatcactgccagggagcaatgcctatagccgtggtccttgtaatctttggtggctgagtatacaacggagctggccttcacactgatctgctggaagaggttccacacttcctgatagatgtattgatttccggtgataaccaggcagcccagctggtcaataatcagcacatcgaggggggagggtggctggcagaatttctgctgtaggatctgcagaatgggctccatgaccttcggggtgtccctcaaggccaccgcaatgtgtcccaaggctcggattgtgtggtcgggaatcaagtgagcgtccaatgccaggtgccccacacgagcctgctgagaacaatgggctgcctctgagagacaggaatag

SEQ ID NO: 18428 - RNA, 3423 nt, Homo sapiens
  source 1..3423: mol_type = other RNA
tgagcaccacacaggccgggcgctcgctcagctgagttgccccaagagttgtgttctgcttgttgtagccagcaaagtgaaggatgctctcagtggccatggccagccccgtgtgctgggacagtcccgatacccagttctgatgtttgttcagatattcctgcaggtgggacttggtgacggtaggtgcccacttcatggcctcctggaggatcatcccacagcgtgcagcgaagtccttcacaatgctctcacgggcttcgtacgtgtcaggaaccgtgatccggtagggggcgtcggggatgtcatagtaaggctgatccttgtgaatatcagcgctcagtgacagtgacagggtctgcaggatgtccagcatggtcttcagcacagtcccgctccagagcaagtggggaaacttatccaccagaccagatagatacttgtctgccaccctccttatcctcttgtggatgtggttgaagttcaccaacaggaactgagcgtgccgctccagctcctcctcgttctccttggtcttggctttatccgccatcatgttcaggaaggcatcgaatactttgtccgcgactgcaatcacacactgcatcatcccagatttgtctttctgaatagctttatcctcaaagtagcagaacattacctggaagcgatcaggatctgttgaacgcagtaccctcatgtactccagccggtacacagagaggaggtaggtggacatggcgaagtccagcttgttgatgagtgcggacacctcgggaggggggtccagcaggttgatgatagtgctgcggagctcactcagctcagcgggggtgaccgtgtcattcttcatggctgagttatactggaggacggaccgcagtggctccttgctgggaaaggtgagcaagggggacttagtggctatttcacagaccccctcgtaccattcttctggccagagtcctgagccctccacagcgaatcccatcagaacggaatacagccagaagtctcggaagagcttctgtaaccgaggcttagcttctttgatgggtggcagtcgtcgggtgagcacagctattacaggaatgagtactcccaagttccctgcactgctagaagcctttagggcagggcccttctcgcttgccctctcgctggctcgcttcccctccagccccagctgcacaaacaactccaacaggttcatgagcagctcatccaccaggtgctcgtcttggatgttggccgcgatgttggccagggcattaatcactgccagggagcaatgcctatagccgtggtccttgtaatctttggtggctgagtatacaacggagctggccttcacactgatctgctggaagaggttccacacttcctgatagatgtattgatttccggtgataaccaggcagcccagctggtcaataatcagcacatcgaggggggagggtggctggcagaatttctgctgtaggatctgcagaatgggctccatgaccttcggggtgtccctcaaggccaccgcaatgtgtcccaaggctcggattgtgtggtcgggaatcaagtgagcgtccttgtcgctctcctgagagatgtagagccggttggacaggctggccaagaacgcctccacaatcactgggtccaccgtcaatccagccttcaggcacctgcagatgttgtcaatagcgatgtctcggagctgctcgtacatggagggctggctcttcttacccgacatgacgttcagggttgactcggaatgctcattggtcacactgatttttatatcattgccagcaactgtgtggtactgactgtggtacttgtagagcttcaccagaactggggacgggatgaccaggaagtctcgcaaggacggtgtcacagagtgcaccaccaccgggaacctctcgcacaggcggcccaaaccctgcagacagcagatcagcaggggcaagtgagcaataatgactttgctggacgtcttggactgcagcttctcagatagcttgatgcaaaggttttctgcaccctgctcgtccttcacagcccacaccatgaggtccacacaggcagcattcgcctgacagcgcagtttgagggggctcagctcattgtggatccggtctgcgtcatgtagaatcttctggagctccccctggctcgtgttgaactgctccagcacaaaatcatggatctccttcacaaaagaggtcgggaggtccttcatgtagtacagagtgtcacgcagcatcttgaacatggtcaggtagagagggtcactgaaggaagtgtagtagagatcagcactggggttggccaggtttaagagttcccgaagcatttccaatggaatgttaaactccttatatgtgacaccgttgaaaaggggagagactgagaagctggagctgatggttgaaaagtagtactcaggctctagggcagtcccatcgggcaagcaggaggcttcaaagtagtgaaaggcagatcctccaggggaactgggagggggcatgccgcgttcagggctgacctgagagatgctggacacactgctggttttcctcttcagggtaccctcctgacagacagtcagcagattgctggggaggatggagcggaagtcattaaaggaacgccttcgaacaccttcaagctcttccaggacacggagggaatgaggagggattttgggaaagagctttgagaggagagactcttccatgttgctgtaacgcccaaatgctcgcgagattcctatcaggcatgggatagcatacttgcaaaggtattctttgtcttgaatctccaaggcctggcacatccccaagaggacatgcaaaacctgcaaaagcacctctaaaatctcatccctaagtgaaggatccctataggccacatcagacagcagagttaccaagcagaagctgaagctctctgcaaccgggagggcacctctgcctttccgagctgtgctttcttctacccaatacacttttggaagacctttgagaagtcgaagaaggtaaggaaccacacaatctttgtgctgaagatcagattcaatcagaaaaatgcccaatgcaatcactgcatctctccgtctttcatctaactggaagatcccatggaaatccactggacacatgcaaagaagcttttggaccttctccaaggatgctggtctctgcaccgccagggagcgggccagtgacaggaccgtgttgaaatagaagccccgcgaggcgctggagccggagccggagcagccgccgccgcctccgcctccgcctccgcctccccgggccggggccgccgccatcacctcacgagccgcggcgctgcccgccggctccccgctcctggcccgcgagcgcccgacctcagggcgcaggcgtaggtgcatcc

SEQ ID NO: 18429 - RNA, 3489 nt, Homo sapiens
  source 1..3489: mol_type = other RNA
tgagcaccacacaggccgggcgctcgctcagctgagttgccccaagagttgtgttctgcttgttgtagccagcaaagtgaaggatgctctcagtggccatggccagccccgtgtgctgggacagtcccgatacccagttctgatgtttgttcagatattcctgcaggtgggacttggtgacggtaggtgcccacttcatggcctcctggaggatcatcccacagcgtgcagcgaagtccttcacaatgctctcacgggcttcgtacgtgtcaggaaccgtgatccggtagggggcgtcggggatgtcatagtaaggctgatccttgtgaatatcagcgctcagtgacagtgacagggtctgcaggatgtccagcatggtcttcagcacagtcccgctccagagcaagtggggaaacttatccaccagaccagatagatacttgtctgccaccctccttatcctcttgtggatgtggttgaagttcaccaacaggaactgagcgtgccgctccagctcctcctcgttctccttggtcttggctttatccgccatcatgttcaggaaggcatcgaatactttgtccgcgactgcaatcacacactgcatcatcccagatttgtctttctgaatagctttatcctcaaagtagcagaacattacctggaagcgatcaggatctgttgaacgcagtaccctcatgtactccagccggtacacagagaggaggtaggtggacatggcgaagtccagcttgttgatgagtgcggacacctcgggaggggggtccagcaggttgatgatagtgctgcggagctcactcagctcagcgggggtgaccgtgtcattcttcatggctgagttatactggaggacggaccgcagtggctccttgctgggaaaggtgagcaagggggacttagtggctatttcacagaccccctcgtaccattcttctggccagagtcctgagccctccacagcgaatcccatcagaacggaatacagccagaagtctcggaagagcttctgtaaccgaggcttagcttctttgatgggtggcagtcgtcgggtgagcacagctattacaggaatgagtactcccaagttccctgcactgctagaagcctttagggcagggcccttctcgcttgccctctcgctggctcgcttcccctccagccccagctgcacaaacaactccaacaggttcatgagcagctcatccaccaggtgctcgtcttggatgttggccgcgatgttggccagggcattaatcactgccagggagcaatgcctatagccgtggtccttgtaatctttggtggctgagtatacaacggagctggccttcacactgatctgctggaagaggttccacacttcctgatagatgtattgatttccggtgataaccaggcagcccagctggtcaataatcagcacatcgaggggggagggtggctggcagaatttctgctgtaggatctgcagaatgggctccatgaccttcggggtgtccctcaaggccaccgcaatgtgtcccaaggctcggattgtgtggtcgggaatcaagtgagcgtccttgtcgctctcctgagagatgtagagccggttggacaggctggccaagaacgcctccacaatcactgggtccaccgtcaatccagccttcaggcacctgcagatgttgtcaatagcgatgtctcggagctgctcgtacatggagggctggctcttcttacccgacatgacgttcagggttgactcggaatgctcattggtcacactgatttttatatcattgccagcaactgtgtggtactgactgtggtacttgtagagcttcaccagaactggggacgggatgaccaggaagtctcgcaaggacggtgtcacagagtgcaccaccaccgggaacctctcgcacaggcggcccaaaccctgcagacagcagatcagcaggggcaagtgagcaataatgactttgctggacgtcttggactgcagcttctcagatagcttgatgcaaaggttttctgcaccctgctcgtccttcacagcccacaccatgaggtccacacaggcagcattcgcctgacagcgcagtttgagggggctcagctcattgtggatccggtctgcgtcatgtagaatcttctggagctccccctggctcgtgttgaactgctccagcacaaaatcatggatctccttcacaaaagaggtcgggaggtccttcatgtagtacagagtgtcacgcagcatcttgaacatggtcaggtagagagggtcactgaaggaagtgtagtagagatcagcactggggttggcctccatcacactggctacaatggcatccaaagatttgagaacagcctcctcaacgatcttcttcaccaggtttaagagttcccgaagcatttccaatggaatgttaaactccttatatgtgacaccgttgaaaaggggagagactgagaagctggagctgatggttgaaaagtagtactcaggctctagggcagtcccatcgggcaagcaggaggcttcaaagtagtgaaaggcagatcctccaggggaactgggagggggcatgccgcgttcagggctgacctgagagatgctggacacactgctggttttcctcttcagggtaccctcctgacagacagtcagcagattgctggggaggatggagcggaagtcattaaaggaacgccttcgaacaccttcaagctcttccaggacacggagggaatgaggagggattttgggaaagagctttgagaggagagactcttccatgttgctgtaacgcccaaatgctcgcgagattcctatcaggcatgggatagcatacttgcaaaggtattctttgtcttgaatctccaaggcctggcacatccccaagaggacatgcaaaacctgcaaaagcacctctaaaatctcatccctaagtgaaggatccctataggccacatcagacagcagagttaccaagcagaagctgaagctctctgcaaccgggagggcacctctgcctttccgagctgtgctttcttctacccaatacacttttggaagacctttgagaagtcgaagaaggtaaggaaccacacaatctttgtgctgaagatcagattcaatcagaaaaatgcccaatgcaatcactgcatctctccgtctttcatctaactggaagatcccatggaaatccactggacacatgcaaagaagcttttggaccttctccaaggatgctggtctctgcaccgccagggagcgggccagtgacaggaccgtgttgaaatagaagccccgcgaggcgctggagccggagccggagcagccgccgccgcctccgcctccgcctccgcctccccgggccggggccgccgccatcacctcacgagccgcggcgctgcccgccggctccccgctcctggcccgcgagcgcccgacctcagggcgcaggcgtaggtgcatcc

SEQ ID NO: 18430 - RNA, 3490 nt, Homo sapiens
  source 1..3490: mol_type = other RNA
tgagcaccacacaggccgggcgctcgctcagctgagttgccccaagagttgtgttctgcttgttgtagccagcaaagtgaaggatgctctcagtggccatggccagccccgtgtgctgggacagtcccgatacccagttctgatgtttgttcagatattcctgcaggtgggacttggtgacggtaggtgcccacttcatggcctcctggaggatcatcccacagcgtgcagcgaagtccttcacaatgctctcacgggcttcgtacgtgtcaggaaccgtgatccggtagggggcgtcggggatgtcatagtaaggctgatccttgtgaatatcagcgctcagtgacagtgacagggtctgcaggatgtccagcatggtcttcagcacagtcccgctccagagcaagtggggaaacttatccaccagaccagatagatacttgtctgccaccctccttatcctcttgtggatgtggttgaagttcaccaacaggaactgagcgtgccgctccagctcctcctcgttctccttggtcttggctttatccgccatcatgttcaggaaggcatcgaatactttgtccgcgactgcaatcacacactgcatcatcccagatttgtctttctgaatagctttatcctcaaagtagcagaacattacctggaagcgatcaggatctgttgaacgcagtaccctcatgtactccagccggtacacagagaggaggtaggtggacatggcgaagtccagcttgttgatgagtgcggacacctcgggaggggggtccagcaggttgatgatagtgctgcggagctcactcagctcagcgggggtgaccgtgtcattcttcatggctgagttatactggaggacggaccgcagtggctccttgctgggaaaggtgagcaagggggacttagtggctatttcacagaccccctcgtaccattcttctggccagagtcctgagccctccacagcgaatcccatcagaacggaatacagccagaagtctcggaagagcttctgtaaccgaggcttagcttctttgatgggtggcagtcgtcgggtgagcacagctattacaggaatgagtactcccaagttccctgcactgctagaagcctttagggcagggcccttctcgcttgccctctcgctggctcgcttcccctccagccccagctgcacaaacaactccaacaggttcatgagcagctcatccaccaggtgctcgtcttggatgttggccgcgatgttggccagggcattaatcactgccagggagcaatgcctatagccgtggtccttgtaatctttggtggctgagtatacaacggagctggccttcacactgatctgctggaagaggttccacacttcctgatagatgtattgatttccggtgataaccaggcagcccagctggtcaataatcagcacatcgaggggggagggtggctggcagaatttctgctgtaggatctgcagaatgggctccatgaccttcggggtgtccctcaaggccaccgcaatgtgtcccaaggctcggattgtgtggtcgggaatcaagtgagcgtccttgtcgctctcctgagagatgtagagccggttggacaggctggccaagaacgcctccacaatcactgggtccaccgtcaatccagccttcaggcacctgcagatgttgtcaatagcgatgtctcggagctgctcgtacatggagggctggctcttcttacccgacatgacgttcagggttgactcggaatgctcattggtcacactgatttttatatcattgccagcaactgtgtggtactgactgtggtacttgtagagcttcaccagaactggggacgggatgaccaggaagtctcgcaaggacggtgtcacagagtgcaccaccaccgggaacctctcgcacaggcggcccaaaccctgcagacagcagatcagcaggggcaagtgagcaataatgactttgctggacgtcttggactgcagcttctcagatagcttgatgcaaaggttttctgcaccctgctcgtccttcacagcccacaccatgaggtccacacaggcagcattcgcctgacagcgcagtttgagggggctcagctcattgtggatccggtctgcgtcatgtagaatcttctggagctccccctggctcgtgttgaactgctccagcacaaaatcatggatctccttcacaaaagaggtcgggaggtccttcatgtagtacagagtgtcacgcagcatcttgaacatggtcaggtagagagggtcactgaaggaagtgtagtagagatcagcactggggttggcctccatcacactggctacaatggcatccaaagatttgagaacagcctcctcaacgatcttcttcaccaggtttaagagttcccgaagcatttccaatggaatgttaaactccttatatgtgacaccgttgaaaaggggagagactgagaagctggagctgatggttgaaaagtagtactcaggctctagggcagtcccatcgggcaagcaggaggcttcaaagtagtgaaaggcagatcctccaggggaactgggagggggcatgccgcgttcagggctgacctgagagatgctggacacactgctggttttcctcttcagggtaccctcctgacagacagtcagcagattgctggggaggatggagcggaagtcattaaaggaacgccttcgaacaccttcaagctcttccaggacacggagggaatgaggagggattttgggaaagagctttgagaggagagactcttccatgttgctgtaacgcccaaatgctcgcgagattcctatcaggcatgggatagcatacttgcaaaggtattctttgtcttgaatctccaaggcctggcacatccccaagaggacatgcaaaacctgcaaaagcacctctaaaatctcatccctaagtgaaggatccctataggccacatcagacagcagagttaccaagcagaagctgaagctctctgcaaccgggagggcacctctgcctttccgagctgtgctttcttctacccaatacacttttggaagacctttgagaagtcgaagaaggtaaggaaccacacaatctttgtgctgaagatcagattcaatcagaaaaatgcccaatgcaatcactgcatctctccgtctttcatctaactggaagatcccatggaaatccactggacacatgcaaagaagcttttggaccttctccaaggatgctggtctctgcaccgccagggagcgggccagtgacaggaccgtgttgaaatagaagccccgcgaggcgctggagccggagccggagcagccgccgccgcctccgcctccgcctccgcctccccgggccggggccgccgccatcacctcacgagccgcggcgctgcccgccggctccccgctcctggcccgcgagcgcccgacctcagggcgcaggcgtaggtgcatccg

SEQ ID NO: 18431 - RNA, 1265 nt, Homo sapiens
  source 1..1265: mol_type = other RNA
tgagcctctccttccctccagcatttgagtcctgtcccaaggcttttcactggcagagcccaaccagaaggcagctgatcacagcctatgaagtgtagtttgcaggcttccacaccccctgttagccagcccctgacttctttcttcccctcaaggcaaaagtagtctctcctatcctttaatctttctttcttcctctgggccctcattgcgtgctgtacatatttgtacacttgtttgtcttgtcacgagcctttctttcctttgtgatgacaggagtcattgtcaaactgaaattccccaactctccaaggaactatgttcaagttcctgaatgtgctttgccctttcttgactttaagcctcttgactttaagtcctctgtccatttctttgttttgttgtttttaatcatctttccaaacagctcaaaatattcttttccaggaatcctttccatactgcctcacatcctttgtactccctcatctgagtatttctctttacaatgaaactttctgcctttttggtctctcacacttgactctgcactcccatgaagggaggagttggagttggattcttggtgttcccagattctggtctgtaaagtaagtatccatggagttaaatggcacagagttgaccagtcagctacatgtcatgtcctggcacatgagctttgtcccgtgctctagggagagagagaaggataaacttttccatctggaccatgaagccagcttaccaacacctgccacttctgggcaatgtgtcctagggatgggtgagccttcttgtatctgcaactttgggtgactgttcctgtttaaagatcttgcagatagggaggtaagtacccaccatccccaggactcaatgccctttccttgccctgggtaacttggctctaagaagtggtgatgaggcttttctcttcccccagtcactgcagaggacacgcttctctacccttctgtctcagaaacgagatctgtctccaactcactcagtcgtttgttttctgggatttggagcagaattaattagcttggaaaaacactaggacaatgctaagtattattaatgacacaacagttccttcctgcaggggatgggtggttcctggttcacttggcagctcttaaagatggacccagttttttccatctttaatctaacaagctctgctccaggccgtgggacactctgtccccagccacttccagtcagggttgttgccaggaactcaattgtatcataat

SEQ ID NO: 18432 - RNA, 4507 nt, Homo sapiens
  source 1..4507: mol_type = other RNA
tgagcctctccttccctccagccccagaggcagctgcctgccttctttttgagttgctttgccgtgattagcactcaggacacagagacggagtattctcactgcctgggagccttggacatacacttgatatagtcctcaatgcagaaaatactgcaaccttgacaacagcagcagcacattagcttgacaaatgcaatcctgccagtagccaagatctctacagttcttccaggcactgggagtccaggacaggaactggatttaacctgcacagtgtagttatttcactgggaacccagatcagggctggggccccagccaacacacttggatatttggcctgcagcgggctggatggtgacgcactaaagcattcctttgcctctacacactccagataaatgaacctcagggtttcatgagttctcaagaaccagcagaaaccaggctctgtcttcttgctatgacccggggtccttatgtgctgggaacaagaggaagtcaatgggtttgggcaggggctgcctggggaagatctcagccaccccgcaggcttatatagagtcctacttccaagctaccctttgggaggaagagtacttgatagatattgcctttaacccaatgcatgggccagagcaacttggggctcagaaaagtacttaaggtggtcaacttatacgcatcatgcacagagcttccttacggaacacacacgaagaggtaaaggctggacagggagaggtggggctggatcaggtcagcataggcgggaggggctgcctctcctgtgttgatcacttcccacctggaggaaaccaagtgaggatgttgtcattgagcgtggcaggaggggacagaaccctcacctgtccagtgcaaaccttctgggtggaaggcagattgcttttagaactaggcctttttatattgccaatgacaaaatcattttcttttttcaaggagtgatgtcaattgtttttcgttctgaatcagtttcaactgcctgaattgcaaattaggatcccaagtgtgggagtgggtagacagagtctgaggacacctcaaggggcctagcctcagaaagcctgaagagcaactcaagtgggtctcacacgggactgagccaagggcccctaggggatcagatcactggggttgggatggaagattggcacccagggcctacccccatccctaggtttagttttataaggcaagtgtttctctcacataaaacaaaaagcaaaacaaatcgcctttgagagtgatctcttttcaccctgtggatcattttgtcttttctttgacataattgcagagaggcgtagagtcccagcttcaagtctaccctcatccaggctccaaggacctaaggttctctctaccttcctttgagttgtcagcaatggtggctgggagtaaggcctgggacagtcttgctgacctgcccccatgaggccacctcccagggcaagcatagcgagggtaggggtgaggctacagtaaagcagggaggtaaagccttatcgtggcgatgctgcagcctgtcccctttcatccgcactgctttagggtaggtcctggacatctctaaatacctagatgctacatcatgccacctctagcttttgtcccctgcagcagctgggtgtgagaaccatttacttttgctttcctgcagcagagagcactgtaggatctgtggcatccctcaatgaatatgttcagaataaaccctgcaatgctctctctgccgccctcctgcatcccctgcaatcagtcttcctttcctcaattattcctaaaacatatctattcatttcattctgttaaaaagtttttttgaatagctctccactgccccacaggttcctcacacacaagcttctcacacagcccccacggtcatgcctgcacctgtcttccccactctccagaggctgccccccacaccacagccacacagaatggggtgatcttccctgattcaccacattctccacacacgcaggtccacctgcttgtgacactgtcctctctgtttgcctggagcaaccctgctcatgctgtgctgaaatgttaccctgacaccttcagagctaacatccctccagttcacagagcacaacacacacacccacagtgcttatctcatgggactctctctctctctctctctctctctctctgggtctttcttcccatcatactgggaatcccaagagcaaaagcatggtgtctagatttacccttatacctccaaccatgtatggtttctggcatgtagtaagtatatgctcaataaaaagttgatgaataaaaaatgatgcaggggtgggaatgggcctagggacttgagagtggcaagtgtttggaagaggtgcttgggggaagtgagtcataaaggtgcccttccctgaagggtgggatttgctgggggaatcatggattagctctctagaatgacagcagaggcttaagaggaacatgtggaatgaatggttgagcactgaagaccaggctgggctcacagactacaatggcacagcaggcaggaactgtggcaaaggacagaaaatggggaggtcaggaaggagctgaacgaggtgtggaaaaaggaataaactaaataggggtgtgagagttcagtggcatcgaaagaagctgggagtggagaagggattgagccgacggtaaaattctggtaacagcacatgctctctcaggcatcatacacaggcaaggcttcaaatgacacagtaggaagaccagcttagaagaaaacctggacagcaactgcatgcccctccctcgggtgttcatttctttttcttctccaggctttcagatcatcgcactgacaaactcaagatgctgaatctgggttgtttaccaaaactgagtacaagttatatcctcaggctcgcttctcaacttccctccctcaggagcagccacaccacaagacactgtgtagcttacagaccattttcaataaattctccttacgaatcattttgcctgattcttctggaagcctcagctgccacagacagttcttttattgtttggtaaccccatggatagcaataaaatcaagatgaaaacacatttgcaaagcaactttcactgtccaaagcacttgcatgtagcattattgaatatttaatactttcatgtaatatttatagagcatcactatgtaccaggcaatgaggatccagtcctgggccccatggaacttacagtctgggagtggaggggcagatgtgatgcaaataatggcaaaaaattgtgactgcagatgatcacaactgtgataagtatatgatggaaaagtacaggacggaggtagcaaggagaccattactttggggagaaacagcaggctccctgaagaagtgacatttaaattgaagagtgagtagaggctatccaggaggtgggcaagggtccataccatgacctcgagaagtctgttgctggaggaatagagagacggctagagagatagattctgctgggccatgggaggccacaggtagaaaaatcaagttgaggaaagaagtggggccagatggggaggacctattgtgctcccctctgagaaagcttgagcaaggggggtcatcattatctgtcctgtgaggacacagaagcttcctggttgggttcgctggagccctggggacagagatcattgcagaccctgctgaaagtctttgcagcccccgtccctctgcagttccactttgtctatgctcagggggtccaggcttggtgccactctgctccattccgtgctcccagtgggatccctcactcgggatggccagctccaggtgtgcttccagggcacagaggacccagggacagaataggacgaagtcactctgaccaccagaaaacagccaagggtaagtcacccttgtagtgctccactaaaaaaagtaaagatgcctatgtgacttgctggaaaacgatgggagaaggcaaaggcccatggaggaagagcttcagggacagccttggctggagaggggaaggggaatctctaaggggaggtgactctagcagggagtacagttgagaacctctggcttaaaaacaaacaaacaaaaaacaccaactctgagctcaagtctgacctctgccacttacagatgctgtgatgttgagcctcagtttcctcgcctgttagctggaattgatgccttccatttttatcccacagggtttttgtaagagttaaaagcaacagctatgaagtcagtgtgaaaagtaaaaataccacacaaaagattgctgaaataatcacatagatcccatttaccttccaaactagacagtaataacaggaaacaatgtacttcatctaacctaggaacatgccattattacctccaccttacacatgggaaaactgaggtatgcactggttaaggaacttgcccaaacatacccatctggaaagtggcagaactgggccccaaaccccagc

SEQ ID NO: 18433 - RNA, 1428 nt, Homo sapiens
  source 1..1428: mol_type = other RNA
tgagcctctccttccctccagctgccatctgccttgggctctatttccgctgtctttagctctggcgagccttggaccagcagcgtgaagttctgggtgcggctgaggaccgggactgtgggcagggaggcctcacatacgtaggtgccattggaatcgaaggtgatagaactgagcgacagcatggggccatcgcccaggggagtggagtccttggtccagcgtagggcaggggtgggcaggccgtgcacggagcagttcacgactgcactgctgtttagaggtaaggaaagcaccttcccctcgctgagctccagggggtccagataggccacgcgcagctccagcgtcttggagagctgcacgtcatctgccgcgtcgtaatcctccactctgcagccataggtcccgctctggccccgggtcactccctccagggtcaagttcccctcgagattcacattcagcacttcctcctgctcatcctgaaggcggaaaagcgtatactccgggctggggctgccgtccccccggcagagcagctggacagtgtcaccctcgcgtacccagcctgctggggtggacgggctgcccacccagaactgcacgtgctccgtgggatagtgcagggtgaggtggaaggtggggctgtccaggcggccgtggcggccctcgggcaggctgtagtgggcggcgcagtggaagctggcgtctcggtcatccttgcggagccgcaggtagagggtgctggtgagggagagcaggcccgaggcctcccggaccgtgcggctggtcatgtagccctctgggttcatctctacgggcacctccaggcgctgcccgttgcgataccacgtgatcttgggggccgggttcccgttccggctgttgcaggtggcgatctcctgggcagagtcctccatcacagacagtgtccctttgttgggggagacctcagtggcctctggctttgcaaacacgttgagccgcgcagtggcctcagcagtgcctgccgcccctgccctcaccacgcacacgtagtctcgctcgtcgcccacctgggcctcagccagcaccaggcgcccctgggagtccagctggtatgggggactgcggccccgggtgtcgtgcattgtgacctggagctcagagccctgcatctcagccgaggctaggcgggggcgagctcccgagcggtcggtaaggaaccattccagcatataatggtcgtgggttcccgtaggggtgcagtccagaatgacagactttcctcgcatcacctccaccagcgggggtacagacaagcgcacctccgcctgggcatctgggtgcgccgccagcaggactgcgagcaacagcagccgcggggccccgcgcgcctgggccggtgcgtccgggggctccatgttcacggcggcggcggagact

SEQ ID NO: 18434 - RNA, 1472 nt, Homo sapiens
  source 1..1472: mol_type = other RNA
tgagcctctccttccctccagctgccatctgccttgggctctatttccgctgtctttagctctggcgagccttggaccagcagcgtgaagttctgggtgcggctgaggaccgggactgtgggcagggaggcctcacatacgtaggtgccattggaatcgaaggtgatagaactgagcgacagcatggggccatcgcccaggggagtggagtccttggtccagcgtagggcaggggtgggcaggccgtgcacggagcagttcacgactgcactgctgtttagaggtaaggaaagcaccttcccctcgctgagctccagggggtccagataggccacgcgcagctccagcgtcttggagagctgcacgtcatctgccgcgtcgtaatcctccactctgcagccataggtcccgctctggccccgggtcactccctccagggtcaagttcccctcgagattcacattcagcacttcctcctgctcatcctgaaggcggaaaagcgtatactccgggctggggctgccgtccccccggcagagcagctggacagtgtcaccctcgcgtacccagcctgctggggtggacgggctgcccacccagaactgcacgtgctccgtgggatagtgcagggtgaggtggaaggtggggctgtccaggcggccgtggcggccctcgggcaggctgtagtgggcggcgcagtggaagctggcgtctcggtcatccttgcggagccgcaggtagagggtgctggtgagggagagcaggcccgaggcctcccggaccgtgcggctggtcatgtagccctctgggttcatctctacgggcacctccaggcgctgcccgttgcgataccacgtgatcttgggggccgggttcccgttccggctgttgcaggtggcgatctcctgggcagagtcctccatcacagacagtgtccctttgttgggggagacctcagtggcctctggctttgcaaacacgttgagccgcgcagtggcctcagcagtgcctgccgcccctgccctcaccacgcacacgtagtctcgctcgtcgcccacctgggcctcagccagcaccaggcgcccctgggagtccagctggtatgggggactgcggccccgggtgtcgtgcattgtgacctggagctcagagccctgcatctcagccgaggctaggcgggggcgagctcccgagcggtcggtaaggaaccattccagcatataatggtcgtgggttcccgtaggggtgcagtccagaatgacagactttcctcgcatcacctccaccagcgggggtacagacaagcgcacctccgcctgggcatctgggtgcgccgccagcaggactgcgagcaacagcagccgcggggccccgcgcgcctgggccggtgcgtccgggggctccatgttcacggcggcggcggagactgagcccgggctgcagctcggccgctgcggggctgggagccagag

SEQ ID NO: 18435 - RNA, 1969 nt, Homo sapiens
  source 1..1969: mol_type = other RNA
tgagcctctccttccctccagggaactcaatggcggagctggcacagggtgtgggcagcggcgggcacaggtgccgtgcggccctgttcaggccaaggtagccaaggacgcccacgagaaggatgctcaggaagctccccagggaggcgaagaagatgagccaatcagaaacctgcacttcgatgctgaagcgctggggctggctccagacacccctcagccacgctgtgtctgctcgcacctgcaccgtgtaggctacaccagcccgcaggccactgagggtaacttgggtctctgtgggctgcacgggatgctctgacacctgtttgctgtcttcatctcggcagcggacaacatactcctttaggacgccgggacaggtgctcagcagggatggtgcccagtccacagacacagagtccaagctatgattcttcaccgagacgtggtgcggtgtcccagctgctgaggcattgcccccaaagtggtaggtggacaggaccgtagaccacaaggtgagcttctcggggtgcgcagaggcaaagatggtaatgtagtaacacttttcctgccccattgccccagactctcgactccagctgtaggttgccattccagccggatccgggtcttgcggcgcagtcaggctgcaggtggcaaggcccccgtcctggcccacaggctgccattcaatgcaatacgtcatgctctgagcccgggctggccaatacatggtggtcccgttggttccgacgctgatattcagagccactggttctgtgtgggtgtcggcaggaatgtgccacgtctggttcaggccaggaccaaattggttcgaggagatgacagccacgttgtaggcagcacccgagagatagggcatcttccccaggtgcagggtcctggtggccttggccttacacgggcaggacagcatgtggagctgtagtcggtaagtgacctccgtgccaggcgccagcccttgacagccttctggaagctccagctgggttggctgctctttcagggtcagccgcctcctcccatcctggcccagctgctccaccgagaatctcacctgaggctgtggggggttttcagggggaacgcacacggggctgctccacttgctccaggaacttccttggctccccagctgccgtcgtcggagctggaattcctgggccacattcatctccagggggcagaggcaggactcagtatcatcatcctgaggtccgcagtcgcccaacttccatgggctgctgggtgtccggtgccggaactgcacctcagcaccaacctggttatccggggtctcccactccatacgcagctgcccggccaacttggacaccttgatgtctcccagaggaggctcatatttaactgagttgtagagctgcagggtcacctcaggagacttctctgtctggttcctggcccaggattccacccagagtgtgacagtgtacagcacagacaccccagcctggtcggagaactgcagcctggtggctgagccggcggcgaagtagcagcagcgcccggagctaaggcaacaccgcaggaagtggctgaccccagctgtgggaccctcatactgccaggagcactcgtaacgatcactggatatccgatagcatctcaggtccctagggcccgaggccgagcctgagtctgcatccggatatggcgggtcctgaaaacagcactcactggttctgcaggcagcgccctgcctggacagcaggaagaggaagaggagggggaccacccaggtcaccagcggctccatcggatccacgtagagccccacagccccaggggagcctctctgccacctgcgaggttcagccaccccgtccccactccggaacacattgaagctgagcaaggagaaaagaccaacgaacatttatggagcgcctgctgtgtgcctggctctggagaggcagcggagtgttct

SEQ ID NO: 18436 - RNA, 2169 nt, Homo sapiens
  source 1..2169: mol_type = other RNA
tgagcctctccttccctccagggaactcaatggcggagctggcacagggtgtgggcagcggcgggcacaggtgccgtgcggccctgttcaggccaaggtagccaaggacgcccacgagaaggatgctcaggaagctccccagggaggcgaagaagatgagccaatcagaaacctgcacttcgatgctgaagcgctggggctggctccagacacccctcagccacgctgtgtctgctcgcacctgcaccgtgtaggctacaccagcccgcaggccactgagggtaacttgggtctctgtgggctgcacgggatgctctgacacctgtttgctgtcttcatctcggcagcggacaacatactcctttaggacgccgggacaggtgctcagcagggatggtgcccagtccacagacacagagtccaagctatgattcttcaccgagacgtggtgcggtgtcccagctgctgaggcattgcccccaaagtggtaggtggacaggaccgtagaccacaaggtgagcttctcggggtgcgcagaggcaaagatggtaatgtagtaacacttttcctgccccattgccccagactctcgactccagctgtaggttgccattccagccggatccgggtcttgcggcgcagtcaggctgcaggtggcaaggcccccgtcctggcccacaggctgccattcaatgcaatacgtcatgctctgagcccgggctggccaatacatggtggtcccgttggttccgacgctgatattcagagccactggttctgtgtgggtgtcggcaggaatgtgccacgtctggttcaggccaggaccaaattggttcgaggagatgacagccacgttgtaggcagcacccgagagatagggcatcttccccaggtgcagggtcctggtggccttggccttacacgggcaggacagcatgtggagctgtagtcggtaagtgacctccgtgccaggcgccagcccttgacagccttctggaagctccagctgggttggctgctctttcagggtcagccgcctcctcccatcctggcccagctgctccaccgagaatctcacctgaggctgtggggggttttcagggggaacgcacacggggctgctccacttgctccaggaacttccttggctccccagctgccgtcgtcggagctggaattcctgggccacattcatctccagggggcagaggcaggactcagtatcatcatcctgaggtccgcagtcgcccaacttccatgggctgctgggtgtccggtgccggaactgcacctcagcaccaacctggttatccggggtctcccactccatacgcagctgcccggccaacttggacaccttgatgtctcccagaggaggctcatatttaactgagttgtagagctgcagggtcacctcaggagacttctctgtctggttcctggcccaggattccacccagagtgtgacagtgtacagcacagacaccccagcctggtcggagaactgcagcctggtggctgagccggcggcgaagtagcagcagcgcccggagctaaggcaacaccgcaggaagtggctgaccccagctgtgggaccctcatactgccaggagcactcgtaacgatcactggatatccgatagcatctcaggtccctagggcccgaggccgagcctgagtctgcatccggatatggcgggtcctgaaaacagcactcactggttctgcaggcagcgccctgcctggacagcaggaagaggaagaggagggggaccacccaggtcaccagcggctccatcggatccacgtagagccccacagccccaggggagcctctctgccacctgcgaggttcagccaccccgtccccactccggaacacattgaagctgagcaaggagaaaagaccaacgaacatttatggagcgcctgctgtgtgcctggctctggagaggcagcggagtgttctgcaacctctggagctgccctcctagaaaccccaacctgttgggggaggtagacgccagagcagcggtgaccccacggagtgatcagttgtgataagggactcacagcaagtgaaggaggcgcctgacccagtcattgctgggagccctggggtagaggaggcagccaagggtggcgaggcattgcagcggggggcggtat

SEQ ID NO: 18437 - RNA, 2171 nt, Homo sapiens
  source 1..2171: mol_type = other RNA
tgagcctctccttccctccagggaactcaatggcggagctggcacagggtgtgggcagcggcgggcacaggtgccgtgcggccctgttcaggccaaggtagccaaggacgcccacgagaaggatgctcaggaagctccccagggaggcgaagaagatgagccaatcagaaacctgcacttcgatgctgaagcgctggggctggctccagacacccctcagccacgctgtgtctgctcgcacctgcaccgtgtaggctacaccagcccgcaggccactgagggtaacttgggtctctgtgggctgcacgggatgctctgacacctgtttgctgtcttcatctcggcagcggacaacatactcctttaggacgccgggacaggtgctcagcagggatggtgcccagtccacagacacagagtccaagctatgattcttcaccgagacgtggtgcggtgtcccagctgctgaggcattgcccccaaagtggtaggtggacaggaccgtagaccacaaggtgagcttctcggggtgcgcagaggcaaagatggtaatgtagtaacacttttcctgccccattgccccagactctcgactccagctgtaggttgccattccagccggatccgggtcttgcggcgcagtcaggctgcaggtggcaaggcccccgtcctggcccacaggctgccattcaatgcaatacgtcatgctctgagcccgggctggccaatacatggtggtcccgttggttccgacgctgatattcagagccactggttctgtgtgggtgtcggcaggaatgtgccacgtctggttcaggccaggaccaaattggttcgaggagatgacagccacgttgtaggcagcacccgagagatagggcatcttccccaggtgcagggtcctggtggccttggccttacacgggcaggacagcatgtggagctgtagtcggtaagtgacctccgtgccaggcgccagcccttgacagccttctggaagctccagctgggttggctgctctttcagggtcagccgcctcctcccatcctggcccagctgctccaccgagaatctcacctgaggctgtggggggttttcagggggaacgcacacggggctgctccacttgctccaggaacttccttggctccccagctgccgtcgtcggagctggaattcctgggccacattcatctccagggggcagaggcaggactcagtatcatcatcctgaggtccgcagtcgcccaacttccatgggctgctgggtgtccggtgccggaactgcacctcagcaccaacctggttatccggggtctcccactccatacgcagctgcccggccaacttggacaccttgatgtctcccagaggaggctcatatttaactgagttgtagagctgcagggtcacctcaggagacttctctgtctggttcctggcccaggattccacccagagtgtgacagtgtacagcacagacaccccagcctggtcggagaactgcagcctggtggctgagccggcggcgaagtagcagcagcgcccggagctaaggcaacaccgcaggaagtggctgaccccagctgtgggaccctcatactgccaggagcactcgtaacgatcactggatatccgatagcatctcaggtccctagggcccgaggccgagcctgagtctgcatccggatatggcgggtcctgaaaacagcactcactggttctgcaggcagcgccctgcctggacagcaggaagaggaagaggagggggaccacccaggtcaccagcggctccatcggatccacgtagagccccacagccccaggggagcctctctgccacctgcgaggttcagccaccccgtccccactccggaacacattgaagctgagcaaggagaaaagaccaacgaacatttatggagcgcctgctgtgtgcctggctctggagaggcagcggagtgttctgcaacctctggagctgccctcctagaaaccccaacctgttgggggaggtagacgccagagcagcggtgaccccacggagtgatcagttgtgataagggactcacagcaagtgaaggaggcgcctgacccagtcattgctgggagccctggggtagaggaggcagccaagggtggcgaggcattgcagcggggggcggtattt

SEQ ID NO: 18438 - RNA, 2172 nt, Homo sapiens
  source 1..2172: mol_type = other RNA
tgagcctctccttccctccagggaactcaatggcggagctggcacagggtgtgggcagcggcgggcacaggtgccgtgcggccctgttcaggccaaggtagccaaggacgcccacgagaaggatgctcaggaagctccccagggaggcgaagaagatgagccaatcagaaacctgcacttcgatgctgaagcgctggggctggctccagacacccctcagccacgctgtgtctgctcgcacctgcaccgtgtaggctacaccagcccgcaggccactgagggtaacttgggtctctgtgggctgcacgggatgctctgacacctgtttgctgtcttcatctcggcagcggacaacatactcctttaggacgccgggacaggtgctcagcagggatggtgcccagtccacagacacagagtccaagctatgattcttcaccgagacgtggtgcggtgtcccagctgctgaggcattgcccccaaagtggtaggtggacaggaccgtagaccacaaggtgagcttctcggggtgcgcagaggcaaagatggtaatgtagtaacacttttcctgccccattgccccagactctcgactccagctgtaggttgccattccagccggatccgggtcttgcggcgcagtcaggctgcaggtggcaaggcccccgtcctggcccacaggctgccattcaatgcaatacgtcatgctctgagcccgggctggccaatacatggtggtcccgttggttccgacgctgatattcagagccactggttctgtgtgggtgtcggcaggaatgtgccacgtctggttcaggccaggaccaaattggttcgaggagatgacagccacgttgtaggcagcacccgagagatagggcatcttccccaggtgcagggtcctggtggccttggccttacacgggcaggacagcatgtggagctgtagtcggtaagtgacctccgtgccaggcgccagcccttgacagccttctggaagctccagctgggttggctgctctttcagggtcagccgcctcctcccatcctggcccagctgctccaccgagaatctcacctgaggctgtggggggttttcagggggaacgcacacggggctgctccacttgctccaggaacttccttggctccccagctgccgtcgtcggagctggaattcctgggccacattcatctccagggggcagaggcaggactcagtatcatcatcctgaggtccgcagtcgcccaacttccatgggctgctgggtgtccggtgccggaactgcacctcagcaccaacctggttatccggggtctcccactccatacgcagctgcccggccaacttggacaccttgatgtctcccagaggaggctcatatttaactgagttgtagagctgcagggtcacctcaggagacttctctgtctggttcctggcccaggattccacccagagtgtgacagtgtacagcacagacaccccagcctggtcggagaactgcagcctggtggctgagccggcggcgaagtagcagcagcgcccggagctaaggcaacaccgcaggaagtggctgaccccagctgtgggaccctcatactgccaggagcactcgtaacgatcactggatatccgatagcatctcaggtccctagggcccgaggccgagcctgagtctgcatccggatatggcgggtcctgaaaacagcactcactggttctgcaggcagcgccctgcctggacagcaggaagaggaagaggagggggaccacccaggtcaccagcggctccatcggatccacgtagagccccacagccccaggggagcctctctgccacctgcgaggttcagccaccccgtccccactccggaacacattgaagctgagcaaggagaaaagaccaacgaacatttatggagcgcctgctgtgtgcctggctctggagaggcagcggagtgttctgcaacctctggagctgccctcctagaaaccccaacctgttgggggaggtagacgccagagcagcggtgaccccacggagtgatcagttgtgataagggactcacagcaagtgaaggaggcgcctgacccagtcattgctgggagccctggggtagaggaggcagccaagggtggcgaggcattgcagcggggggcggtattta

SEQ ID NO: 18439 - RNA, 1909 nt, Homo sapiens
  source 1..1909: mol_type = other RNA
tgagcctctccttccctccagggaactcaatggcggagctggcacagggtgtgggcagcggcgggcacaggtgccgtgcggccctgttcaggccaaggtagccaaggacgcccacgagaaggatgctcaggaagctccccagggaggcgaagaagatgagccaatcagaaacctgcacttcgatgctgaagcgctggggctggctccagacacccctcagccacgctgtgtctgctcgcacctgcaccgtgtaggctacaccagcccgcaggccactgagggtaacttgggtctctgtgggctgcacgggatgctctgacacctgtttgctgtcttcatctcggcagcggacaacatactcctttaggacgccgggacaggtgctcagcagggatggtgcccagtccacagacacagagtccaagctatgattcttcaccgagacgtggtgcggtgtcccagctgctgaggcattgcccccaaagtggtaggtggacaggaccgtagaccacaaggtgagcttctcggggtgcgcagaggcaaagatggtaatgtagtaacacttttcctgccccattgccccagactctcgactccagctgtaggttgccattccagccggatccgggtcttgcggcgcagtcaggctgcaggtggcaaggcccccgtcctggcccacaggctgccattcaatgcaatacgtcatgctctgagcccgggctggccaatacatggtggtcccgttggttccgacgctgatattcagagccactggttctgtgtgggtgtcggcaggaatgtgccacgtctggttcaggccaggaccaaattggttcgaggagatgacagccacgttgtaggcagcacccgagagatagggcatcttccccaggtgcagggtcctggtggccttggccttacacgggcaggacagcatgtggagctgtagtcggtaagtgacctccgtgccaggcgccagcccttgacagccttctggaagctccagctgggttggctgctctttcagggtcagccgcctcctcccatcctggcccagctgctccaccgagaatctcacctgaggctgtggggggttttcagggggaacgcacacggggctgctccacttgctccaggaacttccttggctccccagctgccgtcgtcggagctggaattcctgggccacattcatctccagggggcagaggcaggactcagtatcatcatcctgaggtccgcagtcgcccaacttccatgggctgctgggtgtccggtgccggaactgcacctcagcaccaacctggttatccggggtctcccactccatacgcagctgcccggccaacttggacaccttgatgtctcccagaggaggctcatatttaactgagttgtagagctgcagggtcacctcaggagacttctctgtctggttcctggcccaggattccacccagagtgtgacagtgtacagcacagacaccccagcctggtcggagaactgcagcctggtggctgagccggcggcgaagtagcagcagcgcccggagctaaggcaacaccgcaggaagtggctgaccccagctgtgggaccctcatactgccaggagcactcgtaacgatcactggatatccgatagcatctcaggtccctagggcccgaggccgagcctgagtctgcatccggatatggcgggtcctgaaaacagcactcactggttctgcaggcagcgccctgcctggacagcaggaagaggaagaggagggggaccacccaggtcaccagcggctccatcggatccacgtagagccccacagccccaggggagcctctctgccacctgcgaggttcagccaccccgtccccactccggaacacattgaagctgagcaaggagaaaagact

SEQ ID NO: 18440 - RNA, 2187 nt, Homo sapiens
  source 1..2187: mol_type = other RNA
tgagcctctccttccctccagggaactcaatggcggagctggcacagggtgtgggcagcggcgggcacaggtgccgtgcggccctgttcaggccaaggtagccaaggacgcccacgagaaggatgctcaggaagctccccagggaggcgaagaagatgagccaatcagaaacctgcacttcgatgctgaagcgctggggctggctccagacacccctcagccacgctgtgtctgctcgcacctgcaccgtgtaggctacaccagcccgcaggccactgagggtaacttgggtctctgtgggctgcacgggatgctctgacacctgtttgctgtcttcatctcggcagcggacaacatactcctttaggacgccgggacaggtgctcagcagggatggtgcccagtccacagacacagagtccaagctatgattcttcaccgagacgtggtgcggtgtcccagctgctgaggcattgcccccaaagtggtaggtggacaggaccgtagaccacaaggtgagcttctcggggtgcgcagaggcaaagatggtaatgtagtaacacttttcctgccccattgccccagactctcgactccagctgtaggttgccattccagccggatccgggtcttgcggcgcagtcaggctgcaggtggcaaggcccccgtcctggcccacaggctgccattcaatgcaatacgtcatgctctgagcccgggctggccaatacatggtggtcccgttggttccgacgctgatattcagagccactggttctgtgtgggtgtcggcaggaatgtgccacgtctggttcaggccaggaccaaattggttcgaggagatgacagccacgttgtaggcagcacccgagagatagggcatcttccccaggtgcagggtcctggtggccttggccttacacgggcaggacagcatgtggagctgtagtcggtaagtgacctccgtgccaggcgccagcccttgacagccttctggaagctccagctgggttggctgctctttcagggtcagccgcctcctcccatcctggcccagctgctccaccgagaatctcacctgaggctgtggggggttttcagggggaacgcacacggggctgctccacttgctccaggaacttccttggctccccagctgccgtcgtcggagctggaattcctgggccacattcatctccagggggcagaggcaggactcagtatcatcatcctgaggtccgcagtcgcccaacttccatgggctgctgggtgtccggtgccggaactgcacctcagcaccaacctggttatccggggtctcccactccatacgcagctgcccggccaacttggacaccttgatgtctcccagaggaggctcatatttaactgagttgtagagctgcagggtcacctcaggagacttctctgtctggttcctggcccaggattccacccagagtgtgacagtgtacagcacagacaccccagcctggtcggagaactgcagcctggtggctgagccggcggcgaagtagcagcagcgcccggagctaaggcaacaccgcaggaagtggctgaccccagctgtgggaccctcatactgccaggagcactcgtaacgatcactggatatccgatagcatctcaggtccctagggcccgaggccgagcctggaagagatcctgagtctgcatccggatatggcgggtcctgaaaacagcactcactggttctgcaggcagcgccctgcctggacagcaggaagaggaagaggagggggaccacccaggtcaccagcggctccatcggatccacgtagagccccacagccccaggggagcctctctgccacctgcgaggttcagccaccccgtccccactccggaacacattgaagctgagcaaggagaaaagaccaacgaacatttatggagcgcctgctgtgtgcctggctctggagaggcagcggagtgttctgcaacctctggagctgccctcctagaaaccccaacctgttgggggaggtagacgccagagcagcggtgaccccacggagtgatcagttgtgataagggactcacagcaagtgaaggaggcgcctgacccagtcattgctgggagccctggggtagaggaggcagccaagggtggcgaggcattgcagcggggggcggtatttaggg

SEQ ID NO: 18441 - RNA, 2199 nt, Homo sapiens
  source 1..2199: mol_type = other RNA
tgagcctctccttccctccagggaactcaatggcggagctggcacagggtgtgggcagcggcgggcacaggtgccgtgcggccctgttcaggccaaggtagccaaggacgcccacgagaaggatgctcaggaagctccccagggaggcgaagaagatgagccaatcagaaacctgcacttcgatgctgaagcgctggggctggctccagacacccctcagccacgctgtgtctgctcgcacctgcaccgtgtaggctacaccagcccgcaggccactgagggtaacttgggtctctgtgggctgcacgggatgctctgacacctgtttgctgtcttcatctcggcagcggacaacatactcctttaggacgccgggacaggtgctcagcagggatggtgcccagtccacagacacagagtccaagctatgattcttcaccgagacgtggtgcggtgtcccagctgctgaggcattgcccccaaagtggtaggtggacaggaccgtagaccacaaggtgagcttctcggggtgcgcagaggcaaagatggtaatgtagtaacacttttcctgccccattgccccagactctcgactccagctgtaggttgccattccagccggatccgggtcttgcggcgcagtcaggctgcaggtggcaaggcccccgtcctggcccacaggctgccattcaatgcaatacgtcatgctctgagcccgggctggccaatacatggtggtcccgttggttccgacgctgatattcagagccactggttctgtgtgggtgtcggcaggaatgtgccacgtctggttcaggccaggaccaaattggttcgaggagatgacagccacgttgtaggcagcacccgagagatagggcatcttccccaggtgcagggtcctggtggccttggccttacacgggcaggacagcatgtggagctgtagtcggtaagtgacctccgtgccaggcgccagcccttgacagccttctggaagctccagctgggttggctgctctttcagggtcagccgcctcctcccatcctggcccagctgctccaccgagaatctcacctgaggctgtggggggttttctgcaatcagaaccaaaccaacagggggaacgcacacggggctgctccacttgctccaggaacttccttggctccccagctgccgtcgtcggagctggaattcctgggccacattcatctccagggggcagaggcaggactcagtatcatcatcctgaggtccgcagtcgcccaacttccatgggctgctgggtgtccggtgccggaactgcacctcagcaccaacctggttatccggggtctcccactccatacgcagctgcccggccaacttggacaccttgatgtctcccagaggaggctcatatttaactgagttgtagagctgcagggtcacctcaggagacttctctgtctggttcctggcccaggattccacccagagtgtgacagtgtacagcacagacaccccagcctggtcggagaactgcagcctggtggctgagccggcggcgaagtagcagcagcgcccggagctaaggcaacaccgcaggaagtggctgaccccagctgtgggaccctcatactgccaggagcactcgtaacgatcactggatatccgatagcatctcaggtccctagggcccgaggccgagcctgagtctgcatccggatatggcgggtcctgaaaacagcactcactggttctgcaggcagcgccctgcctggacagcaggaagaggaagaggagggggaccacccaggtcaccagcggctccatcggatccacgtagagccccacagccccaggggagcctctctgccacctgcgaggttcagccaccccgtccccactccggaacacattgaagctgagcaaggagaaaagaccaacgaacatttatggagcgcctgctgtgtgcctggctctggagaggcagcggagtgttctgcaacctctggagctgccctcctagaaaccccaacctgttgggggaggtagacgccagagcagcggtgaccccacggagtgatcagttgtgataagggactcacagcaagtgaaggaggcgcctgacccagtcattgctgggagccctggggtagaggaggcagccaagggtggcgaggcattgcagcggggggcggtatttagggaaa

SEQ ID NO: 18442 - RNA, 1992 nt, Homo sapiens
  source 1..1992: mol_type = other RNA
tgagcctctccttccctccagggaactcaatggcggagctggcacagggtgtgggcagcggcgggcacaggtgccgtgcggccctgttcaggccaaggtagccaaggacgcccacgagaaggatgctcaggaagctccccagggaggcgaagaagatgagccaatcagaaacctgcacttcgatgctgaagcgctggggctggctccagacacccctcagccacgctgtgtctgctcgcacctgcaccgtgtaggctacaccagcccgcaggccactgagggtaacttgggtctctgtgggctgcacgggatgctctgacacctgtttgctgtcttcatctcggcagcggacaacatactcctttaggacgccgggacaggtgctcagcagggatggtgcccagtccacagacacagagtccaagctatgattcttcaccgagacgtggtgcggtgtcccagctgctgaggcattgcccccaaagtggtaggtggacaggaccgtagaccacaaggtgagcttctcggggtgcgcagaggcaaagatggtaatgtagtaacacttttcctgccccattgccccagactctcgactccagctgtaggttgccattccagccggatccgggtcttgcggcgcagtcaggctgcaggtggcaaggcccccgtcctggcccacaggctgccattcaatgcaatacgtcatgctctgagcccgggctggccaatacatggtggtcccgttggttccgacgctgatattcagagccactggttctgtgtgggtgtcggcaggaatgtgccacgtctggttcaggccaggaccaaattggttcgaggagatgacagccacgttgtaggcagcacccgagagatagggcatcttccccaggtgcagggtcctggtggccttggccttacacgggcaggacagcatgtggagctgtagtcggtaagtgacctccgtgccaggcgccagcccttgacagccttctggaagctccagctgggttggctgctctttcagggtcagccgcctcctcccatcctggcccagctgctccaccgagaatctcacctgaggctgtggggggttttctgcaatcagaaccaaaccaacagggggaacgcacacggggctgctccacttgctccaggaacttccttggctccccagctgccgtcgtcggagctggaattcctgggccacattcatctccagggggcagaggcaggactcagtatcatcatcctgaggtccgcagtcgcccaacttccatgggctgctgggtgtccggtgccggaactgcacctcagcaccaacctggttatccggggtctcccactccatacgcagctgcccggccaacttggacaccttgatgtctcccagaggaggctcatatttaactgagttgtagagctgcagggtcacctcaggagacttctctgtctggttcctggcccaggattccacccagagtgtgacagtgtacagcacagacaccccagcctggtcggagaactgcagcctggtggctgagccggcggcgaagtagcagcagcgcccggagctaaggcaacaccgcaggaagtggctgaccccagctgtgggaccctcatactgccaggagcactcgtaacgatcactggatatccgatagcatctcaggtccctagggcccgaggccgagcctgagtctgcatccggatatggcgggtcctgaaaacagcactcactggttctgcaggcagcgccctgcctggacagcaggaagaggaagaggagggggaccacccaggtcaccagcggctccatcggatccacgtagagccccacagccccaggggagcctctctgccacctgcgaggttcagccaccccgtccccactccggaacacattgaagctgagcaaggagaaaagactgaaaaaaaagaaaaaagaaaaaaagtaaagtgtcacagcccatccctaaggcaagtcaaagt

SEQ ID NO: 18443 - RNA, 2211 nt, Homo sapiens
  source 1..2211: mol_type = other RNA
tgagcctctccttccctccagggaactcaatggcggagctggcacagggtgtgggcagcggcgggcacaggtgccgtgcggccctgttcaggccaaggtagccaaggacgcccacgagaaggatgctcaggaagctccccagggaggcgaagaagatgagccaatcagaaacctgcacttcgatgctgaagcgctggggctggctccagacacccctcagccacgctgtgtctgctcgcacctgcaccgtgtaggctacaccagcccgcaggccactgagggtaacttgggtctctgtgggctgcacgggatgctctgacacctgtttgctgtcttcatctcggcagcggacaacatactcctttaggacgccgggacaggtgctcagcagggatggtgcccagtccacagacacagagtccaagctatgattcttcaccgagacgtggtgcggtgtcccagctgctgaggcattgcccccaaagtggtaggtggacaggaccgtagaccacaaggtgagcttctcggggtgcgcagaggcaaagatggtaatgtagtaacacttttcctgccccattgccccagactctcgactccagctgtaggttgccattccagccggatccgggtcttgcggcgcagtcaggctgcaggtggcaaggcccccgtcctggcccacaggctgccattcaatgcaatacgtcatgctctgagcccgggctggccaatacatggtggtcccgttggttccgacgctgatattcagagccactggttctgtgtgggtgtcggcaggaatgtgccacgtctggttcaggccaggaccaaattggttcgaggagatgacagccacgttgtaggcagcacccgagagatagggcatcttccccaggtgcagggtcctggtggccttggccttacacgggcaggacagcatgtggagctgtagtcggtaagtgacctccgtgccaggcgccagcccttgacagccttctggaagctccagctgggttggctgctctttcagggtcagccgcctcctcccatcctggcccagctgctccaccgagaatctcacctgaggctgtggggggttttctgcaatcagaaccaaaccaacagggggaacgcacacggggctgctccacttgctccaggaacttccttggctccccagctgccgtcgtcggagctggaattcctgggccacattcatctccagggggcagaggcaggactcagtatcatcatcctgaggtccgcagtcgcccaacttccatgggctgctgggtgtccggtgccggaactgcacctcagcaccaacctggttatccggggtctcccactccatacgcagctgcccggccaacttggacaccttgatgtctcccagaggaggctcatatttaactgagttgtagagctgcagggtcacctcaggagacttctctgtctggttcctggcccaggattccacccagagtgtgacagtgtacagcacagacaccccagcctggtcggagaactgcagcctggtggctgagccggcggcgaagtagcagcagcgcccggagctaaggcaacaccgcaggaagtggctgaccccagctgtgggaccctcatactgccaggagcactcgtaacgatcactggatatccgatagcatctcaggtccctagggcccgaggccgagcctggaagagatcctgagtctgcatccggatatggcgggtcctgaaaacagcactcactggttctgcaggcagcgccctgcctggacagcaggaagaggaagaggagggggaccacccaggtcaccagcggctccatcggatccacgtagagccccacagccccaggggagcctctctgccacctgcgaggttcagccaccccgtccccactccggaacacattgaagctgagcaaggagaaaagaccaacgaacatttatggagcgcctgctgtgtgcctggctctggagaggcagcggagtgttctgcaacctctggagctgccctcctagaaaccccaacctgttgggggaggtagacgccagagcagcggtgaccccacggagtgatcagttgtgataagggactcacagcaagtgaaggaggcgcctgacccagtcattgctgggagccctggggtagaggaggcagccaagggtggcgaggcattgcagcggggggcggtatttagggaaa

SEQ ID NO: 18444 - RNA, 2212 nt, Homo sapiens
  source 1..2212: mol_type = other RNA
tgagcctctccttccctccagggaactcaatggcggagctggcacagggtgtgggcagcggcgggcacaggtgccgtgcggccctgttcaggccaaggtagccaaggacgcccacgagaaggatgctcaggaagctccccagggaggcgaagaagatgagccaatcagaaacctgcacttcgatgctgaagcgctggggctggctccagacacccctcagccacgctgtgtctgctcgcacctgcaccgtgtaggctacaccagcccgcaggccactgagggtaacttgggtctctgtgggctgcacgggatgctctgacacctgtttgctgtcttcatctcggcagcggacaacatactcctttaggacgccgggacaggtgctcagcagggatggtgcccagtccacagacacagagtccaagctatgattcttcaccgagacgtggtgcggtgtcccagctgctgaggcattgcccccaaagtggtaggtggacaggaccgtagaccacaaggtgagcttctcggggtgcgcagaggcaaagatggtaatgtagtaacacttttcctgccccattgccccagactctcgactccagctgtaggttgccattccagccggatccgggtcttgcggcgcagtcaggctgcaggtggcaaggcccccgtcctggcccacaggctgccattcaatgcaatacgtcatgctctgagcccgggctggccaatacatggtggtcccgttggttccgacgctgatattcagagccactggttctgtgtgggtgtcggcaggaatgtgccacgtctggttcaggccaggaccaaattggttcgaggagatgacagccacgttgtaggcagcacccgagagatagggcatcttccccaggtgcagggtcctggtggccttggccttacacgggcaggacagcatgtggagctgtagtcggtaagtgacctccgtgccaggcgccagcccttgacagccttctggaagctccagctgggttggctgctctttcagggtcagccgcctcctcccatcctggcccagctgctccaccgagaatctcacctgaggctgtggggggttttctgcaatcagaaccaaaccaacagggggaacgcacacggggctgctccacttgctccaggaacttccttggctccccagctgccgtcgtcggagctggaattcctgggccacattcatctccagggggcagaggcaggactcagtatcatcatcctgaggtccgcagtcgcccaacttccatgggctgctgggtgtccggtgccggaactgcacctcagcaccaacctggttatccggggtctcccactccatacgcagctgcccggccaacttggacaccttgatgtctcccagaggaggctcatatttaactgagttgtagagctgcagggtcacctcaggagacttctctgtctggttcctggcccaggattccacccagagtgtgacagtgtacagcacagacaccccagcctggtcggagaactgcagcctggtggctgagccggcggcgaagtagcagcagcgcccggagctaaggcaacaccgcaggaagtggctgaccccagctgtgggaccctcatactgccaggagcactcgtaacgatcactggatatccgatagcatctcaggtccctagggcccgaggccgagcctggaagagatcctgagtctgcatccggatatggcgggtcctgaaaacagcactcactggttctgcaggcagcgccctgcctggacagcaggaagaggaagaggagggggaccacccaggtcaccagcggctccatcggatccacgtagagccccacagccccaggggagcctctctgccacctgcgaggttcagccaccccgtccccactccggaacacattgaagctgagcaaggagaaaagaccaacgaacatttatggagcgcctgctgtgtgcctggctctggagaggcagcggagtgttctgcaacctctggagctgccctcctagaaaccccaacctgttgggggaggtagacgccagagcagcggtgaccccacggagtgatcagttgtgataagggactcacagcaagtgaaggaggcgcctgacccagtcattgctgggagccctggggtagaggaggcagccaagggtggcgaggcattgcagcggggggcggtatttagggaaat

SEQ ID NO: 18445 - RNA, 2213 nt, Homo sapiens
  source 1..2213: mol_type = other RNA
tgagcctctccttccctccagggaactcaatggcggagctggcacagggtgtgggcagcggcgggcacaggtgccgtgcggccctgttcaggccaaggtagccaaggacgcccacgagaaggatgctcaggaagctccccagggaggcgaagaagatgagccaatcagaaacctgcacttcgatgctgaagcgctggggctggctccagacacccctcagccacgctgtgtctgctcgcacctgcaccgtgtaggctacaccagcccgcaggccactgagggtaacttgggtctctgtgggctgcacgggatgctctgacacctgtttgctgtcttcatctcggcagcggacaacatactcctttaggacgccgggacaggtgctcagcagggatggtgcccagtccacagacacagagtccaagctatgattcttcaccgagacgtggtgcggtgtcccagctgctgaggcattgcccccaaagtggtaggtggacaggaccgtagaccacaaggtgagcttctcggggtgcgcagaggcaaagatggtaatgtagtaacacttttcctgccccattgccccagactctcgactccagctgtaggttgccattccagccggatccgggtcttgcggcgcagtcaggctgcaggtggcaaggcccccgtcctggcccacaggctgccattcaatgcaatacgtcatgctctgagcccgggctggccaatacatggtggtcccgttggttccgacgctgatattcagagccactggttctgtgtgggtgtcggcaggaatgtgccacgtctggttcaggccaggaccaaattggttcgaggagatgacagccacgttgtaggcagcacccgagagatagggcatcttccccaggtgcagggtcctggtggccttggccttacacgggcaggacagcatgtggagctgtagtcggtaagtgacctccgtgccaggcgccagcccttgacagccttctggaagctccagctgggttggctgctctttcagggtcagccgcctcctcccatcctggcccagctgctccaccgagaatctcacctgaggctgtggggggttttctgcaatcagaaccaaaccaacagggggaacgcacacggggctgctccacttgctccaggaacttccttggctccccagctgccgtcgtcggagctggaattcctgggccacattcatctccagggggcagaggcaggactcagtatcatcatcctgaggtccgcagtcgcccaacttccatgggctgctgggtgtccggtgccggaactgcacctcagcaccaacctggttatccggggtctcccactccatacgcagctgcccggccaacttggacaccttgatgtctcccagaggaggctcatatttaactgagttgtagagctgcagggtcacctcaggagacttctctgtctggttcctggcccaggattccacccagagtgtgacagtgtacagcacagacaccccagcctggtcggagaactgcagcctggtggctgagccggcggcgaagtagcagcagcgcccggagctaaggcaacaccgcaggaagtggctgaccccagctgtgggaccctcatactgccaggagcactcgtaacgatcactggatatccgatagcatctcaggtccctagggcccgaggccgagcctggaagagatcctgagtctgcatccggatatggcgggtcctgaaaacagcactcactggttctgcaggcagcgccctgcctggacagcaggaagaggaagaggagggggaccacccaggtcaccagcggctccatcggatccacgtagagccccacagccccaggggagcctctctgccacctgcgaggttcagccaccccgtccccactccggaacacattgaagctgagcaaggagaaaagaccaacgaacatttatggagcgcctgctgtgtgcctggctctggagaggcagcggagtgttctgcaacctctggagctgccctcctagaaaccccaacctgttgggggaggtagacgccagagcagcggtgaccccacggagtgatcagttgtgataagggactcacagcaagtgaaggaggcgcctgacccagtcattgctgggagccctggggtagaggaggcagccaagggtggcgaggcattgcagcggggggcggtatttagggaaatg

SEQ ID NO: 18446 - RNA, 2004 nt, Homo sapiens
  source 1..2004: mol_type = other RNA
tgagcctctccttccctccagggaactcaatggcggagctggcacagggtgtgggcagcggcgggcacaggtgccgtgcggccctgttcaggccaaggtagccaaggacgcccacgagaaggatgctcaggaagctccccagggaggcgaagaagatgagccaatcagaaacctgcacttcgatgctgaagcgctggggctggctccagacacccctcagccacgctgtgtctgctcgcacctgcaccgtgtaggctacaccagcccgcaggccactgagggtaacttgggtctctgtgggctgcacgggatgctctgacacctgtttgctgtcttcatctcggcagcggacaacatactcctttaggacgccgggacaggtgctcagcagggatggtgcccagtccacagacacagagtccaagctatgattcttcaccgagacgtggtgcggtgtcccagctgctgaggcattgcccccaaagtggtaggtggacaggaccgtagaccacaaggtgagcttctcggggtgcgcagaggcaaagatggtaatgtagtaacacttttcctgccccattgccccagactctcgactccagctgtaggttgccattccagccggatccgggtcttgcggcgcagtcaggctgcaggtggcaaggcccccgtcctggcccacaggctgccattcaatgcaatacgtcatgctctgagcccgggctggccaatacatggtggtcccgttggttccgacgctgatattcagagccactggttctgtgtgggtgtcggcaggaatgtgccacgtctggttcaggccaggaccaaattggttcgaggagatgacagccacgttgtaggcagcacccgagagatagggcatcttccccaggtgcagggtcctggtggccttggccttacacgggcaggacagcatgtggagctgtagtcggtaagtgacctccgtgccaggcgccagcccttgacagccttctggaagctccagctgggttggctgctctttcagggtcagccgcctcctcccatcctggcccagctgctccaccgagaatctcacctgaggctgtggggggttttctgcaatcagaaccaaaccaacagggggaacgcacacggggctgctccacttgctccaggaacttccttggctccccagctgccgtcgtcggagctggaattcctgggccacattcatctccagggggcagaggcaggactcagtatcatcatcctgaggtccgcagtcgcccaacttccatgggctgctgggtgtccggtgccggaactgcacctcagcaccaacctggttatccggggtctcccactccatacgcagctgcccggccaacttggacaccttgatgtctcccagaggaggctcatatttaactgagttgtagagctgcagggtcacctcaggagacttctctgtctggttcctggcccaggattccacccagagtgtgacagtgtacagcacagacaccccagcctggtcggagaactgcagcctggtggctgagccggcggcgaagtagcagcagcgcccggagctaaggcaacaccgcaggaagtggctgaccccagctgtgggaccctcatactgccaggagcactcgtaacgatcactggatatccgatagcatctcaggtccctagggcccgaggccgagcctggaagagatcctgagtctgcatccggatatggcgggtcctgaaaacagcactcactggttctgcaggcagcgccctgcctggacagcaggaagaggaagaggagggggaccacccaggtcaccagcggctccatcggatccacgtagagccccacagccccaggggagcctctctgccacctgcgaggttcagccaccccgtccccactccggaacacattgaagctgagcaaggagaaaagactgaaaaaaaagaaaaaagaaaaaaagtaaagtgtcacagcccatccctaaggcaagtcaaagt

SEQ ID NO: 18447 - RNA, 1350 nt, Homo sapiens
  source 1..1350: mol_type = other RNA
tgagcctctccttccctccagggaactcaatggcggagctggcacagggtgtgggcagcggcgggcacaggtgccgtgcggccctgttcaggccaaggtagccaaggacgcccacgagaaggatgctcaggaagctccccagggaggcgaagaagatgagccaatcagaaacctgcacttcgatgctgaagcgctggggctggctccagacacccctcagccacgctgtgtctgctcgcacctgcaccgtgtaggctacaccagcccgcaggccactgagggtaacttgggtctctgtgggctgcacgggatgctctgacacctgtttgctgtcttcatctcggcagcggacaacatactcctttaggacgccgggacaggtgctcagcagggatggtgcccagtccacagacacagagtccaagctatgattcttcaccgagacgtggtgcggtgtcccagctgctgaggcattgcccccaaagtggtaggtggacaggaccgtagaccacaaggtgagcttctcggggtgcgcagaggcaaagatggtaatgtagtaacacttttcctgccccattgccccagactctcgactccagctgtaggttgccattccagccggatccgggtcttgcggcgcagtcaggctgcaggtggcaaggcccccgtcctggcccacaggctgccattcaatgcaatacgtcatgctctgagcccgggctggccaatacatggtggtcccgttggttccgacgctgatattcagagccactggttctgtgtgggtgtcggcaggaatgtgccacgtctggttcaggccaggaccaaattggttcgaggagatgacagccacgttgtaggcagcacccgagagatagggcatcttccccaggtgcagggtcctggtggccttggccttacacgggcaggacagcatgtggagctgtagtcggtaagtgacctccgtgccaggcgccagcccttgacagccttctggaagctccagctgggttggctgctctttcagggtcagccgcctcctcccatcctggcccagctgctccaccgagaatctcacctgaggctgtggggggttttctgcaatcagaaccaaaccaacagggggaacgcacacggggctgctccacttgctccaggaacttccttggctccccagctgccgtcgtcggagctggaattcctgggccacattcatctccagggggcagaggcaggactcagtatcatcatcctgaggtccgcagtcgccctgagttgtagagctgcagggtcacctcaggagacttctctgtctggttcctggcccaggattccacccagagtgtgaca

SEQ ID NO: 18448 - RNA, 74 nt, Homo sapiens
  source 1..74: mol_type = other RNA
tgagctaaatgtgtgctgggacatttggctcaaatgtgtcccagcacacatttagctcacctaagacaaataga

SEQ ID NO: 18449 - RNA, 3176 nt, Homo sapiens
  source 1..3176: mol_type = other RNA
tgagctgctgtaccaaaataccacaaactgcatggcttaaaacaacagaaatttattccctcacaatcctggaggccagatgtctgaaatcaagatattggtagggttggttccttctcgagactctgagggagaatctgtgacatgcctgttttcctagcttctagtgacttcctccaattcttagggttctttggctcatagatgcattgctctaatctctgcctccatcttcccatggccttcagctctgtgtgtctatttccccttcttttctaagagctagtcattgaatttagggcccaccctactacaggttgatctcatttccaggtccttgatttcatctgcaaaaactttttccaaataatgtcacacgtggagattcccagtgaatgtatctcctgggggccactattcagcctattacactattcttagaagatgcctagaaggatatggccaatgttatccagaaggcttcatgaaggaggtaatagaagctaacccttcaaagatgaaagttggcgttcattagagggtcacaaggggaggaagggaatgtcaggttcagggaccagccagaccagagctaaggaagtgacatcacatggaacaatttgtgaacagcaagcagtagggcctggctgcaggacagggtgtgaagtgggggagcagtgatcaggagggccagagagatcagcagggatgtgatcttgagaagctgtgtgtgccatgatctggccctattaatccagaagggtctgatggaagcctctgtgattctcttccatggttaaacattttaattgtattatacctcggatattcctaaatatttaaaacactggcatggttgaactagacaacctttaagtagtttgttccaaccatgagatttagatttcatgatttaggttttatgatcttaaactgaaacctgttagttttctaccactagtgagatcatggcctctgcttttctcctgggaagtccctcttataatcactctcttcccatgattaaagggctactctgccttcatgttgctacccgctcccctggaaatggagaatcaagcaaggatgcggttttccttccattactacatccatacaagagtaaatcaagaataaaagtccagttaatgaaaagatcactggtcttaatatacttagcaaaattttaaaggcaattaaaagtatatacatagacaatgatcaaaattctaatgaaaagacccggctctcccctaaaagaagaaaaaatcatgtaatgtatatatgcattccataaaaacatacatggggaaaacttcagaagcctaaaaacaaaacatcagtaaaccaagccacacttagaaaaatgaaagctgatttttattttatcatcaacagccattctttagacatgaacatgcatacgtaatattctacgcacacatcacagcttttaacgttagttaataaaggttaaacacacaacatacatccttacaaaaaaagtcaaaatgcaaacttaaaactttaaacaaaagtattactaatttaaaaaaagtttgtgttgggtaccatttgtacaacacagttaatttaaacattttcattttggttgcacatgaaaaaggcggcagtagaaaataaagtcattgagggtttttaaatagcagaataggcagttttgccatgcaggagaagcaatattaaatattagtttcaaaaaaaatccacatttaaaaatatttagttcaagtcacagaatttttctcagtagagaccccaatgcaatgcataattagctgccttagatggcccgtttgaaaggatgatatcccttcagagtgtaactttactgattttggcacagaaaagaagtcttaagaacatgattaaaaaagagggaagaggaacagaggaaagaaataaaagcaagaataaatgagatagtaattgcaatcactaaaaaactgcattctcagtcattgcagaatactgtcttctgtctacagcaggtgcttattccagaattgttattgcagcatggatttaatttgcttggaggtagtctcatcattcaaatgttttgttgtgtacctgagagcatttagaagaccttccacactattaggaggttggtccttaagaactttgatacaacctttcatatcaattttggaagttttagcaaatgctcccactggatgtacgtggtcatagagtattatgacacccaccattaccctcaagcagaatgacactgtctcttcatttgtaaatctgcttctgtattccggtgtttccagcatgactctgcatacactagccattgtgcttaaacaatctgtggtattttctattggtaaatttttattctctgatacaaattttgttgtggcatcactcaaggttttcagcattggagttgcctcagcataaaacaaagacattcgatttgccaattcattatttacttcattttctccttctgccggtacattgttaatcctcatacgactcaatgttcttctataatagctgaaatcattctgtatggcaggatttgtcatcttgagttcatcaaaccggagtgtgaaatgaagaatttctgcaaactgtttagcaagagcctgctctcgctctagatgctgggtgggagaatatggggtacttgttaaggctcccagaagacctcttaatgctgcttctaacctctgagaaaattcgtaaaatttctttaatttgcctactagtggaacaactgcaccccatgccttctcttgcaacttctcatctgctggatgctggattgcctctcgtatttcgtggccagctcctctgtatgactgcaagtcctccaagatgccttctgcatcttttaatactacattcacctgattataaatttccttctcagactctgtaggctgggcatcaactgggtaaccttgaatgagttaatcaaattccaggcctcagtttcttctcctggcggcccgggcgggcgaggggagcgcggcgcgggagcgcaggagcctcggagcctccggtgccgccgccgccgccgtttccgggttggcggggctcacgtcaccgccacaggtttgcgagctgcccccgccgcggcggcagcagcagcagcagcagcagcccgggcgagtgccaggcgagaaataact

SEQ ID NO: 18450 - RNA, 3076 nt, Homo sapiens
  source 1..3076: mol_type = other RNA
tgagctgctgtaccaaaataccacaaactgcatggcttaaaacaacagaaatttattccctcacaatcctggaggccagatgtctgaaatcaagatattggtagggttggttccttctcgagactctgagggagaatctgtgacatgcctgttttcctagcttctagtgacttcctccaattcttagggttctttggctcatagatgcattgctctaatctctgcctccatcttcccatggccttcagctctgtgtgtctatttccccttcttttctaagagctagtcattgaatttagggcccaccctactacaggttgatctcatttccaggtccttgatttcatctgcaaaaactttttccaaataatgtcacacgtggagattcccagtgaatgtatctcctgggggccactattcagcctattacactattcttagaagatgcctagaaggatatggccaatgttatccagaaggcttcatgaaggaggtaatagaagctaacccttcaaagatgaaagttggcgttcattagagggtcacaaggggaggaagggaatgtcaggttcagggaccagccagaccagagctaaggaagtgacatcacatggaacaatttgtgaacagcaagcagtagggcctggctgcaggacagggtgtgaagtgggggagcagtgatcaggagggccagagagatcagcagggatgtgatcttgagaagctgtgtgtgccatgatctggccctattaatccagaagggtctgatggaagcctctgtgattctcttccatggttaaacattttaattgtattatacctcggatattcctaaatatttaaaacactggcatggttgaactagacaacctttaagtagtttgttccaaccatgagatttagatttcatgatttaggttttatgatcttaaactgaaacctgttagttttctaccactagtgagatcatggcctctgcttttctcctgggaagtccctcttataatcactctcttcccatgattaaagggctactctgccttcatgttgctacccgctcccctggaaatggagaatcaagcaaggatgcggttttccttccattactacatccatacaagagtaaatcaagaataaaagtccagttaatgaaaagatcactggtcttaatatacttagcaaaattttaaaggcaattaaaagtatatacatagacaatgatcaaaattctaatgaaaagacccggctctcccctaaaagaagaaaaaatcatgtaatgtatatatgcattccataaaaacatacatggggaaaacttcagaagcctaaaaacaaaacatcagtaaaccaagccacacttagaaaaatgaaagctgatttttattttatcatcaacagccattctttagacatgaacatgcatacgtaatattctacgcacacatcacagcttttaacgttagttaataaaggttaaacacacaacatacatccttacaaaaaaagtcaaaatgcaaacttaaaactttaaacaaaagtattactaatttaaaaaaagtttgtgttgggtaccatttgtacaacacagttaatttaaacattttcattttggttgcacatgaaaaaggcggcagtagaaaataaagtcattgagggtttttaaatagcagaataggcagttttgccatgcaggagaagcaatattaaatattagtttcaaaaaaaatccacatttaaaaatatttagttcaagtcacagaatttttctcagtagagaccccaatgcaatgcataattagctgccttagatggcccgtttgaaaggatgatatcccttcagagtgtaactttactgattttggcacagaaaagaagtcttaagaacatgattaaaaaagagggaagaggaacagaggaaagaaataaaagcaagaataaatgagatagtaattgcaatcactaaaaaactgcattctcagtcattgcagaatactgtcttctgtctacagcaggtgcttattccagaattgttattgcagcatggatttaatttgcttggaggtagtctcatcattcaaatgttttgttgtgtacctgagagcatttagaagaccttccacactattaggaggttggtccttaagaactttgatacaacctttcatatcaattttggaagttttagcaaatgctcccactggatgtacgtggtcatagagtattatgacacccaccattaccctcaagcagaatgacactgtctcttcatttgtaaatctgcttctgtattccggtgtttccagcatgactctgcatacactagccattgtgcttaaacaatctgtggtattttctattggtaaatttttattctctgatacaaattttgttgtggcatcactcaaggttttcagcattggagttgcctcagcataaaacaaagacattcgatttgccaattcattatttacttcattttctccttctgccggtacattgttaatcctcatacgactcaatgttcttctataatagctgaaatcattctgtatggcaggatttgtcatcttgagttcatcaaaccggagtgtgaaatgaagaatttctgcaaactgtttagcaagagcctgctctcgctctagatgctgggtgggagaatatggggtacttgttaaggctcccagaagacctcttaatgctgcttctaacctctgagaaaattcgtaaaatttctttaatttgcctactagtggaacaactgcaccccatgccttctcttgcaacttctcatctgctggatgctggattgcctctcgtatttcgtggccagctcctctgtatgactgcaagtcctccaagatgccttctgcatcttttaatactacattcacctgattataaatttccttctcagactctgtaggctgggcatcaactgggtaaccttgaatgagttaatcaaattccaggcctcagtttcttctccttcgagaagccgagccgccggcgctcgcacaaaaggaggacgctcgcctcgcgacgcgcctccccccgcgcccagtccccgccgcatcgc

SEQ ID NO: 18451 - RNA, 3123 nt, Homo sapiens
  source 1..3123: mol_type = other RNA
tgagctgctgtaccaaaataccacaaactgcatggcttaaaacaacagaaatttattccctcacaatcctggaggccagatgtctgaaatcaagatattggtagggttggttccttctcgagactctgagggagaatctgtgacatgcctgttttcctagcttctagtgacttcctccaattcttagggttctttggctcatagatgcattgctctaatctctgcctccatcttcccatggccttcagctctgtgtgtctatttccccttcttttctaagagctagtcattgaatttagggcccaccctactacaggttgatctcatttccaggtccttgatttcatctgcaaaaactttttccaaataatgtcacacgtggagattcccagtgaatgtatctcctgggggccactattcagcctattacactattcttagaagatgcctagaaggatatggccaatgttatccagaaggcttcatgaaggaggtaatagaagctaacccttcaaagatgaaagttggcgttcattagagggtcacaaggggaggaagggaatgtcaggttcagggaccagccagaccagagctaaggaagtgacatcacatggaacaatttgtgaacagcaagcagtagggcctggctgcaggacagggtgtgaagtgggggagcagtgatcaggagggccagagagatcagcagggatgtgatcttgagaagctgtgtgtgccatgatctggccctattaatccagaagggtctgatggaagcctctgtgattctcttccatggttaaacattttaattgtattatacctcggatattcctaaatatttaaaacactggcatggttgaactagacaacctttaagtagtttgttccaaccatgagatttagatttcatgatttaggttttatgatcttaaactgaaacctgttagttttctaccactagtgagatcatggcctctgcttttctcctgggaagtccctcttataatcactctcttcccatgattaaagggctactctgccttcatgttgctacccgctcccctggaaatggagaatcaagcaaggatgcggttttccttccattactacatccatacaagagtaaatcaagaataaaagtccagttaatgaaaagatcactggtcttaatatacttagcaaaattttaaaggcaattaaaagtatatacatagacaatgatcaaaattctaatgaaaagacccggctctcccctaaaagaagaaaaaatcatgtaatgtatatatgcattccataaaaacatacatggggaaaacttcagaagcctaaaaacaaaacatcagtaaaccaagccacacttagaaaaatgaaagctgatttttattttatcatcaacagccattctttagacatgaacatgcatacgtaatattctacgcacacatcacagcttttaacgttagttaataaaggttaaacacacaacatacatccttacaaaaaaagtcaaaatgcaaacttaaaactttaaacaaaagtattactaatttaaaaaaagtttgtgttgggtaccatttgtacaacacagttaatttaaacattttcattttggttgcacatgaaaaaggcggcagtagaaaataaagtcattgagggtttttaaatagcagaataggcagttttgccatgcaggagaagcaatattaaatattagtttcaaaaaaaatccacatttaaaaatatttagttcaagtcacagaatttttctcagtagagaccccaatgcaatgcataattagctgccttagatggcccgtttgaaaggatgatatcccttcagagtgtaactttactgattttggcacagaaaagaagtcttaagaacatgattaaaaaagagggaagaggaacagaggaaagaaataaaagcaagaataaatgagatagtaattgcaatcactaaaaaactgcattctcagtcattgcagaatactgtcttctgtctacagcaggtgcttattccagaattgttattgcagcatggatttaatttgcttggaggtagtctcatcattcaaatgttttgttgtgtacctgagagcatttagaagaccttccacactattaggaggttggtccttaagaactttgatacaacctttcatatcaattttggaagttttagcaaatgctcccactggatgtacgtggtcatagagtattatgacacccaccattaccctcaagcagaatgacactgtctcttcatttgtaaatctgcttctgtattccggtgtttccagcatgactctgcatacactagccattgtgcttaaacaatctgtggtattttctattggtaaatttttattctctgatacaaattttgttgtggcatcactcaaggttttcagcattggagttgcctcagcataaaacaaagacattcgatttgccaattcattatttacttcattttctccttctgccggtacattgttaatcctcatacgactcaatgttcttctataatagctgaaatcattctgtatggcaggatttgtcatcttgagttcatcaaaccggagtgtgaaatgaagaatttctgcaaactgtttagcaagagcctgctctcgctctagatgctgggtgggagaatatggggtacttgttaaggctcccagaagacctcttaatgctgcttctaacctctgagaaaattcgtaaaatttctttaatttgcctactagtggaacaactgcaccccatgccttctcttgcaacttctcatctgctggatgctggattgcctctcgtatttcgtggccagctcctctgtatgactgcaagtcctccaagatgccttctgcatcttttaatactacattcacctgattataaatttccttctcagactctgtaggctgggcatctgccactcttcagccagtgctggtgattctgtccttgtccttctatcaactgggtaaccttgaatgagttaatcaaattccaggcctcagtttcttctccttcgagaagccgagccgccggcgctcgcacaaaaggaggacgctcgcctcgcgacgcgcctccccccgcgcccagtccccgccgcatcgc

SEQ ID NO: 18452 - RNA, 3310 nt, Homo sapiens
  source 1..3310: mol_type = other RNA
tgagctgctgtaccaaaataccacaaactgcatggcttaaaacaacagaaatttattccctcacaatcctggaggccagatgtctgaaatcaagatattggtagggttggttccttctcgagactctgagggagaatctgtgacatgcctgttttcctagcttctagtgacttcctccaattcttagggttctttggctcatagatgcattgctctaatctctgcctccatcttcccatggccttcagctctgtgtgtctatttccccttcttttctaagagctagtcattgaatttagggcccaccctactacaggttgatctcatttccaggtccttgatttcatctgcaaaaactttttccaaataatgtcacacgtggagattcccagtgaatgtatctcctgggggccactattcagcctattacactattcttagaagatgcctagaaggatatggccaatgttatccagaaggcttcatgaaggaggtaatagaagctaacccttcaaagatgaaagttggcgttcattagagggtcacaaggggaggaagggaatgtcaggttcagggaccagccagaccagagctaaggaagtgacatcacatggaacaatttgtgaacagcaagcagtagggcctggctgcaggacagggtgtgaagtgggggagcagtgatcaggagggccagagagatcagcagggatgtgatcttgagaagctgtgtgtgccatgatctggccctattaatccagaagggtctgatggaagcctctgtgattctcttccatggttaaacattttaattgtattatacctcggatattcctaaatatttaaaacactggcatggttgaactagacaacctttaagtagtttgttccaaccatgagatttagatttcatgatttaggttttatgatcttaaactgaaacctgttagttttctaccactagtgagatcatggcctctgcttttctcctgggaagtccctcttataatcactctcttcccatgattaaagggctactctgccttcatgttgctacccgctcccctggaaatggagaatcaagcaaggatgcggttttccttccattactacatccatacaagagtaaatcaagaataaaagtccagttaatgaaaagatcactggtcttaatatacttagcaaaattttaaaggcaattaaaagtatatacatagacaatgatcaaaattctaatgaaaagacccggctctcccctaaaagaagaaaaaatcatgtaatgtatatatgcattccataaaaacatacatggggaaaacttcagaagcctaaaaacaaaacatcagtaaaccaagccacacttagaaaaatgaaagctgatttttattttatcatcaacagccattctttagacatgaacatgcatacgtaatattctacgcacacatcacagcttttaacgttagttaataaaggttaaacacacaacatacatccttacaaaaaaagtcaaaatgcaaacttaaaactttaaacaaaagtattactaatttaaaaaaagtttgtgttgggtaccatttgtacaacacagttaatttaaacattttcattttggttgcacatgaaaaaggcggcagtagaaaataaagtcattgagggtttttaaatagcagaataggcagttttgccatgcaggagaagcaatattaaatattagtttcaaaaaaaatccacatttaaaaatatttagttcaagtcacagaatttttctcagtagagaccccaatgcaatgcataattagctgccttagatggcccgtttgaaaggatgatatcccttcagagtgtaactttactgattttggcacagaaaagaagtcttaagaacatgattaaaaaagagggaagaggaacagaggaaagaaataaaagcaagaataaatgagatagtaattgcaatcactaaaaaactgcattctcagtcattgcagaatactgtcttctgtctacagcaggtgcttattccagaattgttattgcagcatggatttaatttgcttggaggtagtctcatcattcaaatgttttgttgtgtacctgagagcatttagaagaccttccacactattaggaggttggtccttaagaactttgatacaacctttcatatcaattttggaagttttagcaaatgctcccactggatgtacgtggtcatagagtattatgacacccaccattaccctcaagcagaatgacactgtctcttcatttgtaaatctgcttctgtattccggtgtttccagcatgactctgcatacactagccattgtgcttaaacaatctgtggtattttctattggtaaatttttattctctgatacaaattttgttgtggcatcactcaaggttttcagcattggagttgcctcagcataaaacaaagacattcgatttgccaattcattatttacttcattttctccttctgccggtacattgttaatcctcatacgactcaatgttcttctataatagctgaaatcattctgtatggcaggatttgtcatcttgagttcatcaaaccggagtgtgaaatgaagaatttctgcaaactgtttagcaagagcctgctctcgctctagatgctgggtgggagaatatggggtacttgttaaggctcccagaagacctcttaatgctgcttctaacctctgagaaaattcgtaaaatttctttaatttgcctactagtggaacaactgcaccccatgccttctcttgcaacttctcatctgctggatgctggattgcctctcgtatttcgtggccagctcctctgtatgactgcaagtcctccaagatgccttctgcatcttttaatactacattcacctgattataaatttccttctcagactctgtaggctgggcatctgccactcttcagccagtgctggtgattctgtccttgtccttctatccttggattggcgttccctctttcctagttcacttgttccagtccttcaacttctgtttcttgctaacaggtgtgcaaatgaattaccaactgggtaaccttgaatgagttaatcaaattccaggcctcagtttcttctcctggcggcccgggcgggcgaggggagcgcggcgcgggagcgcaggagcctcggagcctccggtgccgccgccgccgccgtttccgggttggcggggctcacgtcaccgccacaggtttgcgagctgcccccgccgcggcggcagcagcagcagcagcagcagcccgggcgagtgccaggcgagaaataact

SEQ ID NO: 18453 - RNA, 3210 nt, Homo sapiens
  source 1..3210: mol_type = other RNA
tgagctgctgtaccaaaataccacaaactgcatggcttaaaacaacagaaatttattccctcacaatcctggaggccagatgtctgaaatcaagatattggtagggttggttccttctcgagactctgagggagaatctgtgacatgcctgttttcctagcttctagtgacttcctccaattcttagggttctttggctcatagatgcattgctctaatctctgcctccatcttcccatggccttcagctctgtgtgtctatttccccttcttttctaagagctagtcattgaatttagggcccaccctactacaggttgatctcatttccaggtccttgatttcatctgcaaaaactttttccaaataatgtcacacgtggagattcccagtgaatgtatctcctgggggccactattcagcctattacactattcttagaagatgcctagaaggatatggccaatgttatccagaaggcttcatgaaggaggtaatagaagctaacccttcaaagatgaaagttggcgttcattagagggtcacaaggggaggaagggaatgtcaggttcagggaccagccagaccagagctaaggaagtgacatcacatggaacaatttgtgaacagcaagcagtagggcctggctgcaggacagggtgtgaagtgggggagcagtgatcaggagggccagagagatcagcagggatgtgatcttgagaagctgtgtgtgccatgatctggccctattaatccagaagggtctgatggaagcctctgtgattctcttccatggttaaacattttaattgtattatacctcggatattcctaaatatttaaaacactggcatggttgaactagacaacctttaagtagtttgttccaaccatgagatttagatttcatgatttaggttttatgatcttaaactgaaacctgttagttttctaccactagtgagatcatggcctctgcttttctcctgggaagtccctcttataatcactctcttcccatgattaaagggctactctgccttcatgttgctacccgctcccctggaaatggagaatcaagcaaggatgcggttttccttccattactacatccatacaagagtaaatcaagaataaaagtccagttaatgaaaagatcactggtcttaatatacttagcaaaattttaaaggcaattaaaagtatatacatagacaatgatcaaaattctaatgaaaagacccggctctcccctaaaagaagaaaaaatcatgtaatgtatatatgcattccataaaaacatacatggggaaaacttcagaagcctaaaaacaaaacatcagtaaaccaagccacacttagaaaaatgaaagctgatttttattttatcatcaacagccattctttagacatgaacatgcatacgtaatattctacgcacacatcacagcttttaacgttagttaataaaggttaaacacacaacatacatccttacaaaaaaagtcaaaatgcaaacttaaaactttaaacaaaagtattactaatttaaaaaaagtttgtgttgggtaccatttgtacaacacagttaatttaaacattttcattttggttgcacatgaaaaaggcggcagtagaaaataaagtcattgagggtttttaaatagcagaataggcagttttgccatgcaggagaagcaatattaaatattagtttcaaaaaaaatccacatttaaaaatatttagttcaagtcacagaatttttctcagtagagaccccaatgcaatgcataattagctgccttagatggcccgtttgaaaggatgatatcccttcagagtgtaactttactgattttggcacagaaaagaagtcttaagaacatgattaaaaaagagggaagaggaacagaggaaagaaataaaagcaagaataaatgagatagtaattgcaatcactaaaaaactgcattctcagtcattgcagaatactgtcttctgtctacagcaggtgcttattccagaattgttattgcagcatggatttaatttgcttggaggtagtctcatcattcaaatgttttgttgtgtacctgagagcatttagaagaccttccacactattaggaggttggtccttaagaactttgatacaacctttcatatcaattttggaagttttagcaaatgctcccactggatgtacgtggtcatagagtattatgacacccaccattaccctcaagcagaatgacactgtctcttcatttgtaaatctgcttctgtattccggtgtttccagcatgactctgcatacactagccattgtgcttaaacaatctgtggtattttctattggtaaatttttattctctgatacaaattttgttgtggcatcactcaaggttttcagcattggagttgcctcagcataaaacaaagacattcgatttgccaattcattatttacttcattttctccttctgccggtacattgttaatcctcatacgactcaatgttcttctataatagctgaaatcattctgtatggcaggatttgtcatcttgagttcatcaaaccggagtgtgaaatgaagaatttctgcaaactgtttagcaagagcctgctctcgctctagatgctgggtgggagaatatggggtacttgttaaggctcccagaagacctcttaatgctgcttctaacctctgagaaaattcgtaaaatttctttaatttgcctactagtggaacaactgcaccccatgccttctcttgcaacttctcatctgctggatgctggattgcctctcgtatttcgtggccagctcctctgtatgactgcaagtcctccaagatgccttctgcatcttttaatactacattcacctgattataaatttccttctcagactctgtaggctgggcatctgccactcttcagccagtgctggtgattctgtccttgtccttctatccttggattggcgttccctctttcctagttcacttgttccagtccttcaacttctgtttcttgctaacaggtgtgcaaatgaattaccaactgggtaaccttgaatgagttaatcaaattccaggcctcagtttcttctccttcgagaagccgagccgccggcgctcgcacaaaaggaggacgctcgcctcgcgacgcgcctccccccgcgcccagtccccgccgcatcgc

SEQ ID NO: 18454 - RNA, 3393 nt, Homo sapiens
  source 1..3393: mol_type = other RNA
tgagctgctgtaccaaaataccacaaactgcatggcttaaaacaacagaaatttattccctcacaatcctggaggccagatgtctgaaatcaagatattggtagggttggttccttctcgagactctgagggagaatctgtgacatgcctgttttcctagcttctagtgacttcctccaattcttagggttctttggctcatagatgcattgctctaatctctgcctccatcttcccatggccttcagctctgtgtgtctatttccccttcttttctaagagctagtcattgaatttagggcccaccctactacaggttgatctcatttccaggtccttgatttcatctgcaaaaactttttccaaataatgtcacacgtggagattcccagtgaatgtatctcctgggggccactattcagcctattacactattcttagaagatgcctagaaggatatggccaatgttatccagaaggcttcatgaaggaggtaatagaagctaacccttcaaagatgaaagttggcgttcattagagggtcacaaggggaggaagggaatgtcaggttcagggaccagccagaccagagctaaggaagtgacatcacatggaacaatttgtgaacagcaagcagtagggcctggctgcaggacagggtgtgaagtgggggagcagtgatcaggagggccagagagatcagcagggatgtgatcttgagaagctgtgtgtgccatgatctggccctattaatccagaagggtctgatggaagcctctgtgattctcttccatggttaaacattttaattgtattatacctcggatattcctaaatatttaaaacactggcatggttgaactagacaacctttaagtagtttgttccaaccatgagatttagatttcatgatttaggttttatgatcttaaactgaaacctgttagttttctaccactagtgagatcatggcctctgcttttctcctgggaagtccctcttataatcactctcttcccatgattaaagggctactctgccttcatgttgctacccgctcccctggaaatggagaatcaagcaaggatgcggttttccttccattactacatccatacaagagtaaatcaagaataaaagtccagttaatgaaaagatcactggtcttaatatacttagcaaaattttaaaggcaattaaaagtatatacatagacaatgatcaaaattctaatgaaaagacccggctctcccctaaaagaagaaaaaatcatgtaatgtatatatgcattccataaaaacatacatggggaaaacttcagaagcctaaaaacaaaacatcagtaaaccaagccacacttagaaaaatgaaagctgatttttattttatcatcaacagccattctttagacatgaacatgcatacgtaatattctacgcacacatcacagcttttaacgttagttaataaaggttaaacacacaacatacatccttacaaaaaaagtcaaaatgcaaacttaaaactttaaacaaaagtattactaatttaaaaaaagtttgtgttgggtaccatttgtacaacacagttaatttaaacattttcattttggttgcacatgaaaaaggcggcagtagaaaataaagtcattgagggtttttaaatagcagaataggcagttttgccatgcaggagaagcaatattaaatattagtttcaaaaaaaatccacatttaaaaatatttagttcaagtcacagaatttttctcagtagagaccccaatgcaatgcataattagctgccttagatggcccgtttgaaaggatgatatcccttcagagtgtaactttactgattttggcacagaaaagaagtcttaagaacatgattaaaaaagagggaagaggaacagaggaaagaaataaaagcaagaataaatgagatagtaattgcaatcactaaaaaactgcattctcagtcattgcagaatactgtcttctgtctacagcaggtgcttattccagaattgttattgcagcatggatttaatttgcttggaggtagtctcatcattcaaatgttttgttgtgtacctgagagcatttagaagaccttccacactattaggaggttggtccttaagaactttgatacaacctttcatatcaattttggaagttttagcaaatgctcccactggatgtacgtggtcatagagtattatgacacccaccattaccctcaagcagaatgacactgtctcttcatttgtaaatctgcttctgtattccggtgtttccagcatgactctgcatacactagccattgtgcttaaacaatctgtggtattttctattggtaaatttttattctctgatacaaattttgttgtggcatcactcaaggttttcagcattggagttgcctcagcataaaacaaagacattcgatttgccaattcattatttacttcattttctccttctgccggtacattgttaatcctcatacgactcaatgttcttctataatagctgaaatcattctgtatggcaggatttgtcatcttgagttcatcaaaccggagtgtgaaatgaagaatttctgcaaactgtttagcaagagcctgctctcgctctagatgctgggtgggagaatatggggtacttgttaaggctcccagaagacctcttaatgctgcttctaacctctgagaaaattcgtaaaatttctttaatttgcctactagtggaacaactgcaccccatgccttctcttgcaacttctcatctgctggatgctggattgcctctcgtatttcgtggccagctcctctgtatgactgcaagtcctccaagatgccttctgcatcttttaatactacattcacctgattataaatttccttctcagactctgtaggctgggcatctgccacttttcaaaatcaaggaaaaaatttggcccctgctcaaggtctgtgcatgtcaaaactttaagaagattccccatgttaaggtaccttcagccagtgctggtgattctgtccttgtccttctatccttggattggcgttccctctttcctagttcacttgttccagtccttcaacttctgtttcttgctaacaggtgtgcaaatgaattaccaactgggtaaccttgaatgagttaatcaaattccaggcctcagtttcttctcctggcggcccgggcgggcgaggggagcgcggcgcgggagcgcaggagcctcggagcctccggtgccgccgccgccgccgtttccgggttggcggggctcacgtcaccgccacaggtttgcgagctgcccccgccgcggcggcagcagcagcagcagcagcagcccgggcgagtgccaggcgagaaataact

SEQ ID NO: 18455 - RNA, 3293 nt, Homo sapiens
  source 1..3293: mol_type = other RNA
tgagctgctgtaccaaaataccacaaactgcatggcttaaaacaacagaaatttattccctcacaatcctggaggccagatgtctgaaatcaagatattggtagggttggttccttctcgagactctgagggagaatctgtgacatgcctgttttcctagcttctagtgacttcctccaattcttagggttctttggctcatagatgcattgctctaatctctgcctccatcttcccatggccttcagctctgtgtgtctatttccccttcttttctaagagctagtcattgaatttagggcccaccctactacaggttgatctcatttccaggtccttgatttcatctgcaaaaactttttccaaataatgtcacacgtggagattcccagtgaatgtatctcctgggggccactattcagcctattacactattcttagaagatgcctagaaggatatggccaatgttatccagaaggcttcatgaaggaggtaatagaagctaacccttcaaagatgaaagttggcgttcattagagggtcacaaggggaggaagggaatgtcaggttcagggaccagccagaccagagctaaggaagtgacatcacatggaacaatttgtgaacagcaagcagtagggcctggctgcaggacagggtgtgaagtgggggagcagtgatcaggagggccagagagatcagcagggatgtgatcttgagaagctgtgtgtgccatgatctggccctattaatccagaagggtctgatggaagcctctgtgattctcttccatggttaaacattttaattgtattatacctcggatattcctaaatatttaaaacactggcatggttgaactagacaacctttaagtagtttgttccaaccatgagatttagatttcatgatttaggttttatgatcttaaactgaaacctgttagttttctaccactagtgagatcatggcctctgcttttctcctgggaagtccctcttataatcactctcttcccatgattaaagggctactctgccttcatgttgctacccgctcccctggaaatggagaatcaagcaaggatgcggttttccttccattactacatccatacaagagtaaatcaagaataaaagtccagttaatgaaaagatcactggtcttaatatacttagcaaaattttaaaggcaattaaaagtatatacatagacaatgatcaaaattctaatgaaaagacccggctctcccctaaaagaagaaaaaatcatgtaatgtatatatgcattccataaaaacatacatggggaaaacttcagaagcctaaaaacaaaacatcagtaaaccaagccacacttagaaaaatgaaagctgatttttattttatcatcaacagccattctttagacatgaacatgcatacgtaatattctacgcacacatcacagcttttaacgttagttaataaaggttaaacacacaacatacatccttacaaaaaaagtcaaaatgcaaacttaaaactttaaacaaaagtattactaatttaaaaaaagtttgtgttgggtaccatttgtacaacacagttaatttaaacattttcattttggttgcacatgaaaaaggcggcagtagaaaataaagtcattgagggtttttaaatagcagaataggcagttttgccatgcaggagaagcaatattaaatattagtttcaaaaaaaatccacatttaaaaatatttagttcaagtcacagaatttttctcagtagagaccccaatgcaatgcataattagctgccttagatggcccgtttgaaaggatgatatcccttcagagtgtaactttactgattttggcacagaaaagaagtcttaagaacatgattaaaaaagagggaagaggaacagaggaaagaaataaaagcaagaataaatgagatagtaattgcaatcactaaaaaactgcattctcagtcattgcagaatactgtcttctgtctacagcaggtgcttattccagaattgttattgcagcatggatttaatttgcttggaggtagtctcatcattcaaatgttttgttgtgtacctgagagcatttagaagaccttccacactattaggaggttggtccttaagaactttgatacaacctttcatatcaattttggaagttttagcaaatgctcccactggatgtacgtggtcatagagtattatgacacccaccattaccctcaagcagaatgacactgtctcttcatttgtaaatctgcttctgtattccggtgtttccagcatgactctgcatacactagccattgtgcttaaacaatctgtggtattttctattggtaaatttttattctctgatacaaattttgttgtggcatcactcaaggttttcagcattggagttgcctcagcataaaacaaagacattcgatttgccaattcattatttacttcattttctccttctgccggtacattgttaatcctcatacgactcaatgttcttctataatagctgaaatcattctgtatggcaggatttgtcatcttgagttcatcaaaccggagtgtgaaatgaagaatttctgcaaactgtttagcaagagcctgctctcgctctagatgctgggtgggagaatatggggtacttgttaaggctcccagaagacctcttaatgctgcttctaacctctgagaaaattcgtaaaatttctttaatttgcctactagtggaacaactgcaccccatgccttctcttgcaacttctcatctgctggatgctggattgcctctcgtatttcgtggccagctcctctgtatgactgcaagtcctccaagatgccttctgcatcttttaatactacattcacctgattataaatttccttctcagactctgtaggctgggcatctgccacttttcaaaatcaaggaaaaaatttggcccctgctcaaggtctgtgcatgtcaaaactttaagaagattccccatgttaaggtaccttcagccagtgctggtgattctgtccttgtccttctatccttggattggcgttccctctttcctagttcacttgttccagtccttcaacttctgtttcttgctaacaggtgtgcaaatgaattaccaactgggtaaccttgaatgagttaatcaaattccaggcctcagtttcttctccttcgagaagccgagccgccggcgctcgcacaaaaggaggacgctcgcctcgcgacgcgcctccccccgcgcccagtccccgccgcatcgc

SEQ ID NO: 18456 - RNA, 3459 nt, Homo sapiens
  source 1..3459: mol_type = other RNA
tgagctgctgtaccaaaataccacaaactgcatggcttaaaacaacagaaatttattccctcacaatcctggaggccagatgtctgaaatcaagatattggtagggttggttccttctcgagactctgagggagaatctgtgacatgcctgttttcctagcttctagtgacttcctccaattcttagggttctttggctcatagatgcattgctctaatctctgcctccatcttcccatggccttcagctctgtgtgtctatttccccttcttttctaagagctagtcattgaatttagggcccaccctactacaggttgatctcatttccaggtccttgatttcatctgcaaaaactttttccaaataatgtcacacgtggagattcccagtgaatgtatctcctgggggccactattcagcctattacactattcttagaagatgcctagaaggatatggccaatgttatccagaaggcttcatgaaggaggtaatagaagctaacccttcaaagatgaaagttggcgttcattagagggtcacaaggggaggaagggaatgtcaggttcagggaccagccagaccagagctaaggaagtgacatcacatggaacaatttgtgaacagcaagcagtagggcctggctgcaggacagggtgtgaagtgggggagcagtgatcaggagggccagagagatcagcagggatgtgatcttgagaagctgtgtgtgccatgatctggccctattaatccagaagggtctgatggaagcctctgtgattctcttccatggttaaacattttaattgtattatacctcggatattcctaaatatttaaaacactggcatggttgaactagacaacctttaagtagtttgttccaaccatgagatttagatttcatgatttaggttttatgatcttaaactgaaacctgttagttttctaccactagtgagatcatggcctctgcttttctcctgggaagtccctcttataatcactctcttcccatgattaaagggctactctgccttcatgttgctacccgctcccctggaaatggagaatcaagcaaggatgcggttttccttccattactacatccatacaagagtaaatcaagaataaaagtccagttaatgaaaagatcactggtcttaatatacttagcaaaattttaaaggcaattaaaagtatatacatagacaatgatcaaaattctaatgaaaagacccggctctcccctaaaagaagaaaaaatcatgtaatgtatatatgcattccataaaaacatacatggggaaaacttcagaagcctaaaaacaaaacatcagtaaaccaagccacacttagaaaaatgaaagctgatttttattttatcatcaacagccattctttagacatgaacatgcatacgtaatattctacgcacacatcacagcttttaacgttagttaataaaggttaaacacacaacatacatccttacaaaaaaagtcaaaatgcaaacttaaaactttaaacaaaagtattactaatttaaaaaaagtttgtgttgggtaccatttgtacaacacagttaatttaaacattttcattttggttgcacatgaaaaaggcggcagtagaaaataaagtcattgagggtttttaaatagcagaataggcagttttgccatgcaggagaagcaatattaaatattagtttcaaaaaaaatccacatttaaaaatatttagttcaagtcacagaatttttctcagtagagaccccaatgcaatgcataattagctgccttagatggcccgtttgaaaggatgatatcccttcagagtgtaactttactgattttggcacagaaaagaagtcttaagaacatgattaaaaaagagggaagaggaacagaggaaagaaataaaagcaagaataaatgagatagtaattgcaatcactaaaaaactgcattctcagtcattgcagaatactgtcttctgtctacagcaggtgcttattccagaattgttattgcagcatggatttaatttgcttggaggtagtctcatcattcaaatgttttgttgtgtacctgagagcatttagaagaccttccacactattaggaggttggtccttaagaactttgatacaacctttcatatcaattttggaagttttagcaaatgctcccactggatgtacgtggtcatagagtattatgacacccaccattaccctcaagcagaatgacactgtctcttcatttgtaaatctgcttctgtattccggtgtttccagcatgactctgcatacactagccattgtgcttaaacaatctgtggtattttctattggtaaatttttattctctgatacaaattttgttgtggcatcactcaaggttttcagcattggagttgcctcagcataaaacaaagacattcgatttgccaattcattatttacttcattttctccttctgccggtacattgttaatcctcatacgactcaatgttcttctataatagctgaaatcattctgtatggcaggatttgtcatcttgagttcatcaaaccggagtgtgaaatgaagaatttctgcaaactgtttagcaagagcctgctctcgctctagatgctgggtgggagaatatggggtacttgttaaggctcccagaagacctcttaatgctgcttctaacctctgagaaaattcgtaaaatttctttaatttgcctactagtggaacaactgcaccccatgccttctcttgcaacttctcatctgctggatgctggattgcctctcgtatttcgtggccagctcctctgtatgactgcaagtcctccaagatgccttctgcatcttttaatactacattcacctgattataaatttccttctcagactctgtaggctgggcatctgccacttttcaaaatcaaggaaaaaatttggcccctgctcaaggtctgtgcatgtcaaaactttaagaagattccccatgttaaggtactgccaagtaaacaggccttgtggcagtgaaaggataaactgtccatcattctttcttctcctcggagatttcacaggaaaaggagaaagcgcaggaaacaggaggccttcagccagtgctggtgattctgtccttgtccttctatccttggattggcgttccctctttcctagttcacttgttccagtccttcaacttctgtttcttgctaacaggtgtgcaaatgaattaccctccgctcgagcctccaggcgctctcagtcccgctcctgcgccctcctggagccgcagaggcggctcctcagcggcgctagggggagccccgggtccggagcgggggagcggcggcagccggaccgggagcccctcaacacctgcccctgtggcagagccgcgacaagccaggcggcagctccgagcggggagggcaagtgac

SEQ ID NO: 18457 - RNA, 3376 nt, Homo sapiens
  source 1..3376: mol_type = other RNA
tgagctgctgtaccaaaataccacaaactgcatggcttaaaacaacagaaatttattccctcacaatcctggaggccagatgtctgaaatcaagatattggtagggttggttccttctcgagactctgagggagaatctgtgacatgcctgttttcctagcttctagtgacttcctccaattcttagggttctttggctcatagatgcattgctctaatctctgcctccatcttcccatggccttcagctctgtgtgtctatttccccttcttttctaagagctagtcattgaatttagggcccaccctactacaggttgatctcatttccaggtccttgatttcatctgcaaaaactttttccaaataatgtcacacgtggagattcccagtgaatgtatctcctgggggccactattcagcctattacactattcttagaagatgcctagaaggatatggccaatgttatccagaaggcttcatgaaggaggtaatagaagctaacccttcaaagatgaaagttggcgttcattagagggtcacaaggggaggaagggaatgtcaggttcagggaccagccagaccagagctaaggaagtgacatcacatggaacaatttgtgaacagcaagcagtagggcctggctgcaggacagggtgtgaagtgggggagcagtgatcaggagggccagagagatcagcagggatgtgatcttgagaagctgtgtgtgccatgatctggccctattaatccagaagggtctgatggaagcctctgtgattctcttccatggttaaacattttaattgtattatacctcggatattcctaaatatttaaaacactggcatggttgaactagacaacctttaagtagtttgttccaaccatgagatttagatttcatgatttaggttttatgatcttaaactgaaacctgttagttttctaccactagtgagatcatggcctctgcttttctcctgggaagtccctcttataatcactctcttcccatgattaaagggctactctgccttcatgttgctacccgctcccctggaaatggagaatcaagcaaggatgcggttttccttccattactacatccatacaagagtaaatcaagaataaaagtccagttaatgaaaagatcactggtcttaatatacttagcaaaattttaaaggcaattaaaagtatatacatagacaatgatcaaaattctaatgaaaagacccggctctcccctaaaagaagaaaaaatcatgtaatgtatatatgcattccataaaaacatacatggggaaaacttcagaagcctaaaaacaaaacatcagtaaaccaagccacacttagaaaaatgaaagctgatttttattttatcatcaacagccattctttagacatgaacatgcatacgtaatattctacgcacacatcacagcttttaacgttagttaataaaggttaaacacacaacatacatccttacaaaaaaagtcaaaatgcaaacttaaaactttaaacaaaagtattactaatttaaaaaaagtttgtgttgggtaccatttgtacaacacagttaatttaaacattttcattttggttgcacatgaaaaaggcggcagtagaaaataaagtcattgagggtttttaaatagcagaataggcagttttgccatgcaggagaagcaatattaaatattagtttcaaaaaaaatccacatttaaaaatatttagttcaagtcacagaatttttctcagtagagaccccaatgcaatgcataattagctgccttagatggcccgtttgaaaggatgatatcccttcagagtgtaactttactgattttggcacagaaaagaagtcttaagaacatgattaaaaaagagggaagaggaacagaggaaagaaataaaagcaagaataaatgagatagtaattgcaatcactaaaaaactgcattctcagtcattgcagaatactgtcttctgtctacagcaggtgcttattccagaattgttattgcagcatggatttaatttgcttggaggtagtctcatcattcaaatgttttgttgtgtacctgagagcatttagaagaccttccacactattaggaggttggtccttaagaactttgatacaacctttcatatcaattttggaagttttagcaaatgctcccactggatgtacgtggtcatagagtattatgacacccaccattaccctcaagcagaatgacactgtctcttcatttgtaaatctgcttctgtattccggtgtttccagcatgactctgcatacactagccattgtgcttaaacaatctgtggtattttctattggtaaatttttattctctgatacaaattttgttgtggcatcactcaaggttttcagcattggagttgcctcagcataaaacaaagacattcgatttgccaattcattatttacttcattttctccttctgccggtacattgttaatcctcatacgactcaatgttcttctataatagctgaaatcattctgtatggcaggatttgtcatcttgagttcatcaaaccggagtgtgaaatgaagaatttctgcaaactgtttagcaagagcctgctctcgctctagatgctgggtgggagaatatggggtacttgttaaggctcccagaagacctcttaatgctgcttctaacctctgagaaaattcgtaaaatttctttaatttgcctactagtggaacaactgcaccccatgccttctcttgcaacttctcatctgctggatgctggattgcctctcgtatttcgtggccagctcctctgtatgactgcaagtcctccaagatgccttctgcatcttttaatactacattcacctgattataaatttccttctcagactctgtaggctgggcatctgccacttttcaaaatcaaggaaaaaatttggcccctgctcaaggtctgtgcatgtcaaaactttaagaagattccccatgttaaggtactttcaaagtccaagaaaaaatgtgctgcattgtggtctatgtccctggttagcaccttaatgagattacccatgccagcaaaccttcagccagtgctggtgattctgtccttgtccttctatccttggattggcgttccctctttcctagttcacttgttccagtccttcaacttctgtttcttgctaacaggtgtgcaaatgaattaccaactgggtaaccttgaatgagttaatcaaattccaggcctcagtttcttctccttcgagaagccgagccgccggcgctcgcacaaaaggaggacgctcgcctcgcgacgcgcctccccccgcgcccagtccccgccgcatcgc

SEQ ID NO: 18458 - RNA, 3436 nt, Homo sapiens
  source 1..3436: mol_type = other RNA
tgagctgctgtaccaaaataccacaaactgcatggcttaaaacaacagaaatttattccctcacaatcctggaggccagatgtctgaaatcaagatattggtagggttggttccttctcgagactctgagggagaatctgtgacatgcctgttttcctagcttctagtgacttcctccaattcttagggttctttggctcatagatgcattgctctaatctctgcctccatcttcccatggccttcagctctgtgtgtctatttccccttcttttctaagagctagtcattgaatttagggcccaccctactacaggttgatctcatttccaggtccttgatttcatctgcaaaaactttttccaaataatgtcacacgtggagattcccagtgaatgtatctcctgggggccactattcagcctattacactattcttagaagatgcctagaaggatatggccaatgttatccagaaggcttcatgaaggaggtaatagaagctaacccttcaaagatgaaagttggcgttcattagagggtcacaaggggaggaagggaatgtcaggttcagggaccagccagaccagagctaaggaagtgacatcacatggaacaatttgtgaacagcaagcagtagggcctggctgcaggacagggtgtgaagtgggggagcagtgatcaggagggccagagagatcagcagggatgtgatcttgagaagctgtgtgtgccatgatctggccctattaatccagaagggtctgatggaagcctctgtgattctcttccatggttaaacattttaattgtattatacctcggatattcctaaatatttaaaacactggcatggttgaactagacaacctttaagtagtttgttccaaccatgagatttagatttcatgatttaggttttatgatcttaaactgaaacctgttagttttctaccactagtgagatcatggcctctgcttttctcctgggaagtccctcttataatcactctcttcccatgattaaagggctactctgccttcatgttgctacccgctcccctggaaatggagaatcaagcaaggatgcggttttccttccattactacatccatacaagagtaaatcaagaataaaagtccagttaatgaaaagatcactggtcttaatatacttagcaaaattttaaaggcaattaaaagtatatacatagacaatgatcaaaattctaatgaaaagacccggctctcccctaaaagaagaaaaaatcatgtaatgtatatatgcattccataaaaacatacatggggaaaacttcagaagcctaaaaacaaaacatcagtaaaccaagccacacttagaaaaatgaaagctgatttttattttatcatcaacagccattctttagacatgaacatgcatacgtaatattctacgcacacatcacagcttttaacgttagttaataaaggttaaacacacaacatacatccttacaaaaaaagtcaaaatgcaaacttaaaactttaaacaaaagtattactaatttaaaaaaagtttgtgttgggtaccatttgtacaacacagttaatttaaacattttcattttggttgcacatgaaaaaggcggcagtagaaaataaagtcattgagggtttttaaatagcagaataggcagttttgccatgcaggagaagcaatattaaatattagtttcaaaaaaaatccacatttaaaaatatttagttcaagtcacagaatttttctcagtagagaccccaatgcaatgcataattagctgccttagatggcccgtttgaaaggatgatatcccttcagagtgtaactttactgattttggcacagaaaagaagtcttaagaacatgattaaaaaagagggaagaggaacagaggaaagaaataaaagcaagaataaatgagatagtaattgcaatcactaaaaaactgcattctcagtcattgcagaatactgtcttctgtctacagcaggtgcttattccagaattgttattgcagcatggatttaatttgcttggaggtagtctcatcattcaaatgttttgttgtgtacctgagagcatttagaagaccttccacactattaggaggttggtccttaagaactttgatacaacctttcatatcaattttggaagttttagcaaatgctcccactggatgtacgtggtcatagagtattatgacacccaccattaccctcaagcagaatgacactgtctcttcatttgtaaatctgcttctgtattccggtgtttccagcatgactctgcatacactagccattgtgcttaaacaatctgtggtattttctattggtaaatttttattctctgatacaaattttgttgtggcatcactcaaggttttcagcattggagttgcctcagcataaaacaaagacattcgatttgccaattcattatttacttcattttctccttctgccggtacattgttaatcctcatacgactcaatgttcttctataatagctgaaatcattctgtatggcaggatttgtcatcttgagttcatcaaaccggagtgtgaaatgaagaatttctgcaaactgtttagcaagagcctgctctcgctctagatgctgggtgggagaatatggggtacttgttaaggctcccagaagacctcttaatgctgcttctaacctctgagaaaattcgtaaaatttctttaatttgcctactagtggaacaactgcaccccatgccttctcttgcaacttctcatctgctggatgctggattgcctctcgtatttcgtggccagctcctctgtatgactgcaagtcctccaagatgccttctgcatcttttaatactacattcacctgattataaatttccttctcagactctgtaggctgggcatctgccacttttcaaaatcaaggaaaaaatttggcccctgctcaaggtctgtgcatgtcaaaactttaagaagattccccatgttaaggtactttcaaagtccaagaaaaaatgtgctgcattgtggtctatgtccctggttagcaccttaatgagattacccatgccagcaaaccttcagccagtgctggtgattctgtccttgtccttctatccttggattggcgttccctctttcctagttcacttgttccagtccttcaacttctgtttcttgctaacaggtgtgcaaatgaattaccctccgctcgagcctccaggcgctctcagtcccgctcctgcgccctcctggagccgcagaggcggctcctcagcggcgctagggggagccccgggtccggagcgggggagcggcggcagccggaccgggagcccctcaacacctgcccctgtggcagagccgcgacaagccaggcggcagctccgagcggggagggcaagtgac

SEQ ID NO: 18459 - RNA, 3215 nt, Homo sapiens
  source 1..3215: mol_type = other RNA
tgagctgctgtaccaaaataccacaaactgcatggcttaaaacaacagaaatttattccctcacaatcctggaggccagatgtctgaaatcaagatattggtagggttggttccttctcgagactctgagggagaatctgtgacatgcctgttttcctagcttctagtgacttcctccaattcttagggttctttggctcatagatgcattgctctaatctctgcctccatcttcccatggccttcagctctgtgtgtctatttccccttcttttctaagagctagtcattgaatttagggcccaccctactacaggttgatctcatttccaggtccttgatttcatctgcaaaaactttttccaaataatgtcacacgtggagattcccagtgaatgtatctcctgggggccactattcagcctattacactattcttagaagatgcctagaaggatatggccaatgttatccagaaggcttcatgaaggaggtaatagaagctaacccttcaaagatgaaagttggcgttcattagagggtcacaaggggaggaagggaatgtcaggttcagggaccagccagaccagagctaaggaagtgacatcacatggaacaatttgtgaacagcaagcagtagggcctggctgcaggacagggtgtgaagtgggggagcagtgatcaggagggccagagagatcagcagggatgtgatcttgagaagctgtgtgtgccatgatctggccctattaatccagaagggtctgatggaagcctctgtgattctcttccatggttaaacattttaattgtattatacctcggatattcctaaatatttaaaacactggcatggttgaactagacaacctttaagtagtttgttccaaccatgagatttagatttcatgatttaggttttatgatcttaaactgaaacctgttagttttctaccactagtgagatcatggcctctgcttttctcctgggaagtccctcttataatcactctcttcccatgattaaagggctactctgccttcatgttgctacccgctcccctggaaatggagaatcaagcaaggatgcggttttccttccattactacatccatacaagagtaaatcaagaataaaagtccagttaatgaaaagatcactggtcttaatatacttagcaaaattttaaaggcaattaaaagtatatacatagacaatgatcaaaattctaatgaaaagacccggctctcccctaaaagaagaaaaaatcatgtaatgtatatatgcattccataaaaacatacatggggaaaacttcagaagcctaaaaacaaaacatcagtaaaccaagccacacttagaaaaatgaaagctgatttttattttatcatcaacagccattctttagacatgaacatgcatacgtaatattctacgcacacatcacagcttttaacgttagttaataaaggttaaacacacaacatacatccttacaaaaaaagtcaaaatgcaaacttaaaactttaaacaaaagtattactaatttaaaaaaagtttgtgttgggtaccatttgtacaacacagttaatttaaacattttcattttggttgcacatgaaaaaggcggcagtagaaaataaagtcattgagggtttttaaatagcagaataggcagttttgccatgcaggagaagcaatattaaatattagtttcaaaaaaaatccacatttaaaaatatttagttcaagtcacagaatttttctcagtagagaccccaatgcaatgcataattagctgccttagatggcccgtttgaaaggatgatatcccttcagagtgtaactttactgattttggcacagaaaagaagtcttaagaacatgattaaaaaagagggaagaggaacagaggaaagaaataaaagcaagaataaatgagatagtaattgcaatcactaaaaaactgcattctcagtcattgcagaatactgtcttctgtctacagcaggtgcttattccagaattgttattgcagcatggatttaatttgcttggaggtagtctcatcattcaaatgttttgttgtgtacctgagagcatttagaagaccttccacactattaggaggttggtccttaagaactttgatacaacctttcatatcaattttggaagttttagcaaatgctcccactggatgtacgtggtcatagagtattatgacacccaccattaccctcaagcagaatgacactgtctcttcatttgtaaatctgcttctgtattccggtgtttccagcatgactctgcatacactagccattgtgcttaaacaatctgtggtattttctattggtaaatttttattctctgatacaaattttgttgtggcatcactcaaggttttcagcattggagttgcctcagcataaaacaaagacattcgatttgccaattcattatttacttcattttctccttctgccggtacattgttaatcctcatacgactcaatgttcttctataatagctgaaatcattctgtatggcaggatttgtcatcttgagttcatcaaaccggagtgtgaaatgaagaatttctgcaaactgtttagcaagagcctgctctcgctctagatgctgggtgggagaatatggggtacttgttaaggctcccagaagacctcttaatgctgcttctaacctctgagaaaattcgtaaaatttctttaatttgcctactagtggaacaactgcaccccatgccttctcttgcaacttctcatctgctggatgctggattgcctctcgtatttcgtggccagctcctctgtatgactgcaagtcctccaagatgccttctgcatcttttaatactacattcacctgattataaatttccttctcagactctgtaggctgggcatcttcagccagtgctggtgattctgtccttgtccttctatcaactgggtaaccttgaatgagttaatcaaattccaggcctcagtttcttctcctggcggcccgggcgggcgaggggagcgcggcgcgggagcgcaggagcctcggagcctccggtgccgccgccgccgccgtttccgggttggcggggctcacgtcaccgccacaggtttgcgagctgcccccgccgcggcggcagcagcagcagcagcagcagcccgggcgagtgccaggcgagaaataact

SEQ ID NO: 18460 - RNA, 3115 nt, Homo sapiens
  source 1..3115: mol_type = other RNA
tgagctgctgtaccaaaataccacaaactgcatggcttaaaacaacagaaatttattccctcacaatcctggaggccagatgtctgaaatcaagatattggtagggttggttccttctcgagactctgagggagaatctgtgacatgcctgttttcctagcttctagtgacttcctccaattcttagggttctttggctcatagatgcattgctctaatctctgcctccatcttcccatggccttcagctctgtgtgtctatttccccttcttttctaagagctagtcattgaatttagggcccaccctactacaggttgatctcatttccaggtccttgatttcatctgcaaaaactttttccaaataatgtcacacgtggagattcccagtgaatgtatctcctgggggccactattcagcctattacactattcttagaagatgcctagaaggatatggccaatgttatccagaaggcttcatgaaggaggtaatagaagctaacccttcaaagatgaaagttggcgttcattagagggtcacaaggggaggaagggaatgtcaggttcagggaccagccagaccagagctaaggaagtgacatcacatggaacaatttgtgaacagcaagcagtagggcctggctgcaggacagggtgtgaagtgggggagcagtgatcaggagggccagagagatcagcagggatgtgatcttgagaagctgtgtgtgccatgatctggccctattaatccagaagggtctgatggaagcctctgtgattctcttccatggttaaacattttaattgtattatacctcggatattcctaaatatttaaaacactggcatggttgaactagacaacctttaagtagtttgttccaaccatgagatttagatttcatgatttaggttttatgatcttaaactgaaacctgttagttttctaccactagtgagatcatggcctctgcttttctcctgggaagtccctcttataatcactctcttcccatgattaaagggctactctgccttcatgttgctacccgctcccctggaaatggagaatcaagcaaggatgcggttttccttccattactacatccatacaagagtaaatcaagaataaaagtccagttaatgaaaagatcactggtcttaatatacttagcaaaattttaaaggcaattaaaagtatatacatagacaatgatcaaaattctaatgaaaagacccggctctcccctaaaagaagaaaaaatcatgtaatgtatatatgcattccataaaaacatacatggggaaaacttcagaagcctaaaaacaaaacatcagtaaaccaagccacacttagaaaaatgaaagctgatttttattttatcatcaacagccattctttagacatgaacatgcatacgtaatattctacgcacacatcacagcttttaacgttagttaataaaggttaaacacacaacatacatccttacaaaaaaagtcaaaatgcaaacttaaaactttaaacaaaagtattactaatttaaaaaaagtttgtgttgggtaccatttgtacaacacagttaatttaaacattttcattttggttgcacatgaaaaaggcggcagtagaaaataaagtcattgagggtttttaaatagcagaataggcagttttgccatgcaggagaagcaatattaaatattagtttcaaaaaaaatccacatttaaaaatatttagttcaagtcacagaatttttctcagtagagaccccaatgcaatgcataattagctgccttagatggcccgtttgaaaggatgatatcccttcagagtgtaactttactgattttggcacagaaaagaagtcttaagaacatgattaaaaaagagggaagaggaacagaggaaagaaataaaagcaagaataaatgagatagtaattgcaatcactaaaaaactgcattctcagtcattgcagaatactgtcttctgtctacagcaggtgcttattccagaattgttattgcagcatggatttaatttgcttggaggtagtctcatcattcaaatgttttgttgtgtacctgagagcatttagaagaccttccacactattaggaggttggtccttaagaactttgatacaacctttcatatcaattttggaagttttagcaaatgctcccactggatgtacgtggtcatagagtattatgacacccaccattaccctcaagcagaatgacactgtctcttcatttgtaaatctgcttctgtattccggtgtttccagcatgactctgcatacactagccattgtgcttaaacaatctgtggtattttctattggtaaatttttattctctgatacaaattttgttgtggcatcactcaaggttttcagcattggagttgcctcagcataaaacaaagacattcgatttgccaattcattatttacttcattttctccttctgccggtacattgttaatcctcatacgactcaatgttcttctataatagctgaaatcattctgtatggcaggatttgtcatcttgagttcatcaaaccggagtgtgaaatgaagaatttctgcaaactgtttagcaagagcctgctctcgctctagatgctgggtgggagaatatggggtacttgttaaggctcccagaagacctcttaatgctgcttctaacctctgagaaaattcgtaaaatttctttaatttgcctactagtggaacaactgcaccccatgccttctcttgcaacttctcatctgctggatgctggattgcctctcgtatttcgtggccagctcctctgtatgactgcaagtcctccaagatgccttctgcatcttttaatactacattcacctgattataaatttccttctcagactctgtaggctgggcatcttcagccagtgctggtgattctgtccttgtccttctatcaactgggtaaccttgaatgagttaatcaaattccaggcctcagtttcttctccttcgagaagccgagccgccggcgctcgcacaaaaggaggacgctcgcctcgcgacgcgcctccccccgcgcccagtccccgccgcatcgc

SEQ ID NO: 18461 - RNA, 3175 nt, Homo sapiens
  source 1..3175: mol_type = other RNA
tgagctgctgtaccaaaataccacaaactgcatggcttaaaacaacagaaatttattccctcacaatcctggaggccagatgtctgaaatcaagatattggtagggttggttccttctcgagactctgagggagaatctgtgacatgcctgttttcctagcttctagtgacttcctccaattcttagggttctttggctcatagatgcattgctctaatctctgcctccatcttcccatggccttcagctctgtgtgtctatttccccttcttttctaagagctagtcattgaatttagggcccaccctactacaggttgatctcatttccaggtccttgatttcatctgcaaaaactttttccaaataatgtcacacgtggagattcccagtgaatgtatctcctgggggccactattcagcctattacactattcttagaagatgcctagaaggatatggccaatgttatccagaaggcttcatgaaggaggtaatagaagctaacccttcaaagatgaaagttggcgttcattagagggtcacaaggggaggaagggaatgtcaggttcagggaccagccagaccagagctaaggaagtgacatcacatggaacaatttgtgaacagcaagcagtagggcctggctgcaggacagggtgtgaagtgggggagcagtgatcaggagggccagagagatcagcagggatgtgatcttgagaagctgtgtgtgccatgatctggccctattaatccagaagggtctgatggaagcctctgtgattctcttccatggttaaacattttaattgtattatacctcggatattcctaaatatttaaaacactggcatggttgaactagacaacctttaagtagtttgttccaaccatgagatttagatttcatgatttaggttttatgatcttaaactgaaacctgttagttttctaccactagtgagatcatggcctctgcttttctcctgggaagtccctcttataatcactctcttcccatgattaaagggctactctgccttcatgttgctacccgctcccctggaaatggagaatcaagcaaggatgcggttttccttccattactacatccatacaagagtaaatcaagaataaaagtccagttaatgaaaagatcactggtcttaatatacttagcaaaattttaaaggcaattaaaagtatatacatagacaatgatcaaaattctaatgaaaagacccggctctcccctaaaagaagaaaaaatcatgtaatgtatatatgcattccataaaaacatacatggggaaaacttcagaagcctaaaaacaaaacatcagtaaaccaagccacacttagaaaaatgaaagctgatttttattttatcatcaacagccattctttagacatgaacatgcatacgtaatattctacgcacacatcacagcttttaacgttagttaataaaggttaaacacacaacatacatccttacaaaaaaagtcaaaatgcaaacttaaaactttaaacaaaagtattactaatttaaaaaaagtttgtgttgggtaccatttgtacaacacagttaatttaaacattttcattttggttgcacatgaaaaaggcggcagtagaaaataaagtcattgagggtttttaaatagcagaataggcagttttgccatgcaggagaagcaatattaaatattagtttcaaaaaaaatccacatttaaaaatatttagttcaagtcacagaatttttctcagtagagaccccaatgcaatgcataattagctgccttagatggcccgtttgaaaggatgatatcccttcagagtgtaactttactgattttggcacagaaaagaagtcttaagaacatgattaaaaaagagggaagaggaacagaggaaagaaataaaagcaagaataaatgagatagtaattgcaatcactaaaaaactgcattctcagtcattgcagaatactgtcttctgtctacagcaggtgcttattccagaattgttattgcagcatggatttaatttgcttggaggtagtctcatcattcaaatgttttgttgtgtacctgagagcatttagaagaccttccacactattaggaggttggtccttaagaactttgatacaacctttcatatcaattttggaagttttagcaaatgctcccactggatgtacgtggtcatagagtattatgacacccaccattaccctcaagcagaatgacactgtctcttcatttgtaaatctgcttctgtattccggtgtttccagcatgactctgcatacactagccattgtgcttaaacaatctgtggtattttctattggtaaatttttattctctgatacaaattttgttgtggcatcactcaaggttttcagcattggagttgcctcagcataaaacaaagacattcgatttgccaattcattatttacttcattttctccttctgccggtacattgttaatcctcatacgactcaatgttcttctataatagctgaaatcattctgtatggcaggatttgtcatcttgagttcatcaaaccggagtgtgaaatgaagaatttctgcaaactgtttagcaagagcctgctctcgctctagatgctgggtgggagaatatggggtacttgttaaggctcccagaagacctcttaatgctgcttctaacctctgagaaaattcgtaaaatttctttaatttgcctactagtggaacaactgcaccccatgccttctcttgcaacttctcatctgctggatgctggattgcctctcgtatttcgtggccagctcctctgtatgactgcaagtcctccaagatgccttctgcatcttttaatactacattcacctgattataaatttccttctcagactctgtaggctgggcatcttcagccagtgctggtgattctgtccttgtccttctatcctccgctcgagcctccaggcgctctcagtcccgctcctgcgccctcctggagccgcagaggcggctcctcagcggcgctagggggagccccgggtccggagcgggggagcggcggcagccggaccgggagcccctcaacacctgcccctgtggcagagccgcgacaagccaggcggcagctccgagcggggagggcaagtgac

SEQ ID NO: 18462 - RNA, 3223 nt, Homo sapiens
  source 1..3223: mol_type = other RNA
tgagctgctgtaccaaaataccacaaactgcatggcttaaaacaacagaaatttattccctcacaatcctggaggccagatgtctgaaatcaagatattggtagggttggttccttctcgagactctgagggagaatctgtgacatgcctgttttcctagcttctagtgacttcctccaattcttagggttctttggctcatagatgcattgctctaatctctgcctccatcttcccatggccttcagctctgtgtgtctatttccccttcttttctaagagctagtcattgaatttagggcccaccctactacaggttgatctcatttccaggtccttgatttcatctgcaaaaactttttccaaataatgtcacacgtggagattcccagtgaatgtatctcctgggggccactattcagcctattacactattcttagaagatgcctagaaggatatggccaatgttatccagaaggcttcatgaaggaggtaatagaagctaacccttcaaagatgaaagttggcgttcattagagggtcacaaggggaggaagggaatgtcaggttcagggaccagccagaccagagctaaggaagtgacatcacatggaacaatttgtgaacagcaagcagtagggcctggctgcaggacagggtgtgaagtgggggagcagtgatcaggagggccagagagatcagcagggatgtgatcttgagaagctgtgtgtgccatgatctggccctattaatccagaagggtctgatggaagcctctgtgattctcttccatggttaaacattttaattgtattatacctcggatattcctaaatatttaaaacactggcatggttgaactagacaacctttaagtagtttgttccaaccatgagatttagatttcatgatttaggttttatgatcttaaactgaaacctgttagttttctaccactagtgagatcatggcctctgcttttctcctgggaagtccctcttataatcactctcttcccatgattaaagggctactctgccttcatgttgctacccgctcccctggaaatggagaatcaagcaaggatgcggttttccttccattactacatccatacaagagtaaatcaagaataaaagtccagttaatgaaaagatcactggtcttaatatacttagcaaaattttaaaggcaattaaaagtatatacatagacaatgatcaaaattctaatgaaaagacccggctctcccctaaaagaagaaaaaatcatgtaatgtatatatgcattccataaaaacatacatggggaaaacttcagaagcctaaaaacaaaacatcagtaaaccaagccacacttagaaaaatgaaagctgatttttattttatcatcaacagccattctttagacatgaacatgcatacgtaatattctacgcacacatcacagcttttaacgttagttaataaaggttaaacacacaacatacatccttacaaaaaaagtcaaaatgcaaacttaaaactttaaacaaaagtattactaatttaaaaaaagtttgtgttgggtaccatttgtacaacacagttaatttaaacattttcattttggttgcacatgaaaaaggcggcagtagaaaataaagtcattgagggtttttaaatagcagaataggcagttttgccatgcaggagaagcaatattaaatattagtttcaaaaaaaatccacatttaaaaatatttagttcaagtcacagaatttttctcagtagagaccccaatgcaatgcataattagctgccttagatggcccgtttgaaaggatgatatcccttcagagtgtaactttactgattttggcacagaaaagaagtcttaagaacatgattaaaaaagagggaagaggaacagaggaaagaaataaaagcaagaataaatgagatagtaattgcaatcactaaaaaactgcattctcagtcattgcagaatactgtcttctgtctacagcaggtgcttattccagaattgttattgcagcatggatttaatttgcttggaggtagtctcatcattcaaatgttttgttgtgtacctgagagcatttagaagaccttccacactattaggaggttggtccttaagaactttgatacaacctttcatatcaattttggaagttttagcaaatgctcccactggatgtacgtggtcatagagtattatgacacccaccattaccctcaagcagaatgacactgtctcttcatttgtaaatctgcttctgtattccggtgtttccagcatgactctgcatacactagccattgtgcttaaacaatctgtggtattttctattggtaaatttttattctctgatacaaattttgttgtggcatcactcaaggttttcagcattggagttgcctcagcataaaacaaagacattcgatttgccaattcattatttacttcattttctccttctgccggtacattgttaatcctcatacgactcaatgttcttctataatagctgaaatcattctgtatggcaggatttgtcatcttgagttcatcaaaccggagtgtgaaatgaagaatttctgcaaactgtttagcaagagcctgctctcgctctagatgctgggtgggagaatatggggtacttgttaaggctcccagaagacctcttaatgctgcttctaacctctgagaaaattcgtaaaatttctttaatttgcctactagtggaacaactgcaccccatgccttctcttgcaacttctcatctgctggatgctggattgcctctcgtatttcgtggccagctcctctgtatgactgcaagtcctccaagatgccttctgcatcttttaatactacattcacctgattataaatttccttctcagactctgtaggctgggcatcttcagccagtgctggtgattctgtccttgtccttctatccttggattggcgttccctctttcctagttcacttgttccagtccttcaacttctgtttcttgctaacaggtgtgcaaatgaattaccaactgggtaaccttgaatgagttaatcaaattccaggcctcagtttcttctcctggacttcaggaatggtgacagcccctgcctggctcacctcgcagcggggtcagtgagaggaatgctgtccacgcacccattcagccctcccgcagatacttactgggcct

SEQ ID NO: 18463 - RNA, 3302 nt, Homo sapiens
  source 1..3302: mol_type = other RNA
tgagctgctgtaccaaaataccacaaactgcatggcttaaaacaacagaaatttattccctcacaatcctggaggccagatgtctgaaatcaagatattggtagggttggttccttctcgagactctgagggagaatctgtgacatgcctgttttcctagcttctagtgacttcctccaattcttagggttctttggctcatagatgcattgctctaatctctgcctccatcttcccatggccttcagctctgtgtgtctatttccccttcttttctaagagctagtcattgaatttagggcccaccctactacaggttgatctcatttccaggtccttgatttcatctgcaaaaactttttccaaataatgtcacacgtggagattcccagtgaatgtatctcctgggggccactattcagcctattacactattcttagaagatgcctagaaggatatggccaatgttatccagaaggcttcatgaaggaggtaatagaagctaacccttcaaagatgaaagttggcgttcattagagggtcacaaggggaggaagggaatgtcaggttcagggaccagccagaccagagctaaggaagtgacatcacatggaacaatttgtgaacagcaagcagtagggcctggctgcaggacagggtgtgaagtgggggagcagtgatcaggagggccagagagatcagcagggatgtgatcttgagaagctgtgtgtgccatgatctggccctattaatccagaagggtctgatggaagcctctgtgattctcttccatggttaaacattttaattgtattatacctcggatattcctaaatatttaaaacactggcatggttgaactagacaacctttaagtagtttgttccaaccatgagatttagatttcatgatttaggttttatgatcttaaactgaaacctgttagttttctaccactagtgagatcatggcctctgcttttctcctgggaagtccctcttataatcactctcttcccatgattaaagggctactctgccttcatgttgctacccgctcccctggaaatggagaatcaagcaaggatgcggttttccttccattactacatccatacaagagtaaatcaagaataaaagtccagttaatgaaaagatcactggtcttaatatacttagcaaaattttaaaggcaattaaaagtatatacatagacaatgatcaaaattctaatgaaaagacccggctctcccctaaaagaagaaaaaatcatgtaatgtatatatgcattccataaaaacatacatggggaaaacttcagaagcctaaaaacaaaacatcagtaaaccaagccacacttagaaaaatgaaagctgatttttattttatcatcaacagccattctttagacatgaacatgcatacgtaatattctacgcacacatcacagcttttaacgttagttaataaaggttaaacacacaacatacatccttacaaaaaaagtcaaaatgcaaacttaaaactttaaacaaaagtattactaatttaaaaaaagtttgtgttgggtaccatttgtacaacacagttaatttaaacattttcattttggttgcacatgaaaaaggcggcagtagaaaataaagtcattgagggtttttaaatagcagaataggcagttttgccatgcaggagaagcaatattaaatattagtttcaaaaaaaatccacatttaaaaatatttagttcaagtcacagaatttttctcagtagagaccccaatgcaatgcataattagctgccttagatggcccgtttgaaaggatgatatcccttcagagtgtaactttactgattttggcacagaaaagaagtcttaagaacatgattaaaaaagagggaagaggaacagaggaaagaaataaaagcaagaataaatgagatagtaattgcaatcactaaaaaactgcattctcagtcattgcagaatactgtcttctgtctacagcaggtgcttattccagaattgttattgcagcatggatttaatttgcttggaggtagtctcatcattcaaatgttttgttgtgtacctgagagcatttagaagaccttccacactattaggaggttggtccttaagaactttgatacaacctttcatatcaattttggaagttttagcaaatgctcccactggatgtacgtggtcatagagtattatgacacccaccattaccctcaagcagaatgacactgtctcttcatttgtaaatctgcttctgtattccggtgtttccagcatgactctgcatacactagccattgtgcttaaacaatctgtggtattttctattggtaaatttttattctctgatacaaattttgttgtggcatcactcaaggttttcagcattggagttgcctcagcataaaacaaagacattcgatttgccaattcattatttacttcattttctccttctgccggtacattgttaatcctcatacgactcaatgttcttctataatagctgaaatcattctgtatggcaggatttgtcatcttgagttcatcaaaccggagtgtgaaatgaagaatttctgcaaactgtttagcaagagcctgctctcgctctagatgctgggtgggagaatatggggtacttgttaaggctcccagaagacctcttaatgctgcttctaacctctgagaaaattcgtaaaatttctttaatttgcctactagtggaacaactgcaccccatgccttctcttgcaacttctcatctgctggatgctggattgcctctcgtatttcgtggccagctcctctgtatgactgcaagtcctccaagatgccttctgcatcttttaatactacattcacctgattataaatttccttctcagactctgtaggctgggcatcttcagccagtgctggtgattctgtccttgtccttctatccttggattggcgttccctctttcctagttcacttgttccagtccttcaacttctgtttcttgctaacaggtgtgcaaatgaattaccaactgggtaaccttgaatgagttaatcaaattccaggcctcagtttcttctcctggcggcccgggcgggcgaggggagcgcggcgcgggagcgcaggagcctcggagcctccggtgccgccgccgccgccgtttccgggttggcggggctcacgtcaccgccacaggtttgcgagctgcccccgccgcggcggcagcagcagcagcagcagcagcccgggcgagtgccaggcgagaaataact

SEQ ID NO: 18464 - RNA, 3202 nt, Homo sapiens
  source 1..3202: mol_type = other RNA
tgagctgctgtaccaaaataccacaaactgcatggcttaaaacaacagaaatttattccctcacaatcctggaggccagatgtctgaaatcaagatattggtagggttggttccttctcgagactctgagggagaatctgtgacatgcctgttttcctagcttctagtgacttcctccaattcttagggttctttggctcatagatgcattgctctaatctctgcctccatcttcccatggccttcagctctgtgtgtctatttccccttcttttctaagagctagtcattgaatttagggcccaccctactacaggttgatctcatttccaggtccttgatttcatctgcaaaaactttttccaaataatgtcacacgtggagattcccagtgaatgtatctcctgggggccactattcagcctattacactattcttagaagatgcctagaaggatatggccaatgttatccagaaggcttcatgaaggaggtaatagaagctaacccttcaaagatgaaagttggcgttcattagagggtcacaaggggaggaagggaatgtcaggttcagggaccagccagaccagagctaaggaagtgacatcacatggaacaatttgtgaacagcaagcagtagggcctggctgcaggacagggtgtgaagtgggggagcagtgatcaggagggccagagagatcagcagggatgtgatcttgagaagctgtgtgtgccatgatctggccctattaatccagaagggtctgatggaagcctctgtgattctcttccatggttaaacattttaattgtattatacctcggatattcctaaatatttaaaacactggcatggttgaactagacaacctttaagtagtttgttccaaccatgagatttagatttcatgatttaggttttatgatcttaaactgaaacctgttagttttctaccactagtgagatcatggcctctgcttttctcctgggaagtccctcttataatcactctcttcccatgattaaagggctactctgccttcatgttgctacccgctcccctggaaatggagaatcaagcaaggatgcggttttccttccattactacatccatacaagagtaaatcaagaataaaagtccagttaatgaaaagatcactggtcttaatatacttagcaaaattttaaaggcaattaaaagtatatacatagacaatgatcaaaattctaatgaaaagacccggctctcccctaaaagaagaaaaaatcatgtaatgtatatatgcattccataaaaacatacatggggaaaacttcagaagcctaaaaacaaaacatcagtaaaccaagccacacttagaaaaatgaaagctgatttttattttatcatcaacagccattctttagacatgaacatgcatacgtaatattctacgcacacatcacagcttttaacgttagttaataaaggttaaacacacaacatacatccttacaaaaaaagtcaaaatgcaaacttaaaactttaaacaaaagtattactaatttaaaaaaagtttgtgttgggtaccatttgtacaacacagttaatttaaacattttcattttggttgcacatgaaaaaggcggcagtagaaaataaagtcattgagggtttttaaatagcagaataggcagttttgccatgcaggagaagcaatattaaatattagtttcaaaaaaaatccacatttaaaaatatttagttcaagtcacagaatttttctcagtagagaccccaatgcaatgcataattagctgccttagatggcccgtttgaaaggatgatatcccttcagagtgtaactttactgattttggcacagaaaagaagtcttaagaacatgattaaaaaagagggaagaggaacagaggaaagaaataaaagcaagaataaatgagatagtaattgcaatcactaaaaaactgcattctcagtcattgcagaatactgtcttctgtctacagcaggtgcttattccagaattgttattgcagcatggatttaatttgcttggaggtagtctcatcattcaaatgttttgttgtgtacctgagagcatttagaagaccttccacactattaggaggttggtccttaagaactttgatacaacctttcatatcaattttggaagttttagcaaatgctcccactggatgtacgtggtcatagagtattatgacacccaccattaccctcaagcagaatgacactgtctcttcatttgtaaatctgcttctgtattccggtgtttccagcatgactctgcatacactagccattgtgcttaaacaatctgtggtattttctattggtaaatttttattctctgatacaaattttgttgtggcatcactcaaggttttcagcattggagttgcctcagcataaaacaaagacattcgatttgccaattcattatttacttcattttctccttctgccggtacattgttaatcctcatacgactcaatgttcttctataatagctgaaatcattctgtatggcaggatttgtcatcttgagttcatcaaaccggagtgtgaaatgaagaatttctgcaaactgtttagcaagagcctgctctcgctctagatgctgggtgggagaatatggggtacttgttaaggctcccagaagacctcttaatgctgcttctaacctctgagaaaattcgtaaaatttctttaatttgcctactagtggaacaactgcaccccatgccttctcttgcaacttctcatctgctggatgctggattgcctctcgtatttcgtggccagctcctctgtatgactgcaagtcctccaagatgccttctgcatcttttaatactacattcacctgattataaatttccttctcagactctgtaggctgggcatcttcagccagtgctggtgattctgtccttgtccttctatccttggattggcgttccctctttcctagttcacttgttccagtccttcaacttctgtttcttgctaacaggtgtgcaaatgaattaccaactgggtaaccttgaatgagttaatcaaattccaggcctcagtttcttctccttcgagaagccgagccgccggcgctcgcacaaaaggaggacgctcgcctcgcgacgcgcctccccccgcgcccagtccccgccgcatcgc

SEQ ID NO: 18465 - RNA, 3262 nt, Homo sapiens
  source 1..3262: mol_type = other RNA
tgagctgctgtaccaaaataccacaaactgcatggcttaaaacaacagaaatttattccctcacaatcctggaggccagatgtctgaaatcaagatattggtagggttggttccttctcgagactctgagggagaatctgtgacatgcctgttttcctagcttctagtgacttcctccaattcttagggttctttggctcatagatgcattgctctaatctctgcctccatcttcccatggccttcagctctgtgtgtctatttccccttcttttctaagagctagtcattgaatttagggcccaccctactacaggttgatctcatttccaggtccttgatttcatctgcaaaaactttttccaaataatgtcacacgtggagattcccagtgaatgtatctcctgggggccactattcagcctattacactattcttagaagatgcctagaaggatatggccaatgttatccagaaggcttcatgaaggaggtaatagaagctaacccttcaaagatgaaagttggcgttcattagagggtcacaaggggaggaagggaatgtcaggttcagggaccagccagaccagagctaaggaagtgacatcacatggaacaatttgtgaacagcaagcagtagggcctggctgcaggacagggtgtgaagtgggggagcagtgatcaggagggccagagagatcagcagggatgtgatcttgagaagctgtgtgtgccatgatctggccctattaatccagaagggtctgatggaagcctctgtgattctcttccatggttaaacattttaattgtattatacctcggatattcctaaatatttaaaacactggcatggttgaactagacaacctttaagtagtttgttccaaccatgagatttagatttcatgatttaggttttatgatcttaaactgaaacctgttagttttctaccactagtgagatcatggcctctgcttttctcctgggaagtccctcttataatcactctcttcccatgattaaagggctactctgccttcatgttgctacccgctcccctggaaatggagaatcaagcaaggatgcggttttccttccattactacatccatacaagagtaaatcaagaataaaagtccagttaatgaaaagatcactggtcttaatatacttagcaaaattttaaaggcaattaaaagtatatacatagacaatgatcaaaattctaatgaaaagacccggctctcccctaaaagaagaaaaaatcatgtaatgtatatatgcattccataaaaacatacatggggaaaacttcagaagcctaaaaacaaaacatcagtaaaccaagccacacttagaaaaatgaaagctgatttttattttatcatcaacagccattctttagacatgaacatgcatacgtaatattctacgcacacatcacagcttttaacgttagttaataaaggttaaacacacaacatacatccttacaaaaaaagtcaaaatgcaaacttaaaactttaaacaaaagtattactaatttaaaaaaagtttgtgttgggtaccatttgtacaacacagttaatttaaacattttcattttggttgcacatgaaaaaggcggcagtagaaaataaagtcattgagggtttttaaatagcagaataggcagttttgccatgcaggagaagcaatattaaatattagtttcaaaaaaaatccacatttaaaaatatttagttcaagtcacagaatttttctcagtagagaccccaatgcaatgcataattagctgccttagatggcccgtttgaaaggatgatatcccttcagagtgtaactttactgattttggcacagaaaagaagtcttaagaacatgattaaaaaagagggaagaggaacagaggaaagaaataaaagcaagaataaatgagatagtaattgcaatcactaaaaaactgcattctcagtcattgcagaatactgtcttctgtctacagcaggtgcttattccagaattgttattgcagcatggatttaatttgcttggaggtagtctcatcattcaaatgttttgttgtgtacctgagagcatttagaagaccttccacactattaggaggttggtccttaagaactttgatacaacctttcatatcaattttggaagttttagcaaatgctcccactggatgtacgtggtcatagagtattatgacacccaccattaccctcaagcagaatgacactgtctcttcatttgtaaatctgcttctgtattccggtgtttccagcatgactctgcatacactagccattgtgcttaaacaatctgtggtattttctattggtaaatttttattctctgatacaaattttgttgtggcatcactcaaggttttcagcattggagttgcctcagcataaaacaaagacattcgatttgccaattcattatttacttcattttctccttctgccggtacattgttaatcctcatacgactcaatgttcttctataatagctgaaatcattctgtatggcaggatttgtcatcttgagttcatcaaaccggagtgtgaaatgaagaatttctgcaaactgtttagcaagagcctgctctcgctctagatgctgggtgggagaatatggggtacttgttaaggctcccagaagacctcttaatgctgcttctaacctctgagaaaattcgtaaaatttctttaatttgcctactagtggaacaactgcaccccatgccttctcttgcaacttctcatctgctggatgctggattgcctctcgtatttcgtggccagctcctctgtatgactgcaagtcctccaagatgccttctgcatcttttaatactacattcacctgattataaatttccttctcagactctgtaggctgggcatcttcagccagtgctggtgattctgtccttgtccttctatccttggattggcgttccctctttcctagttcacttgttccagtccttcaacttctgtttcttgctaacaggtgtgcaaatgaattaccctccgctcgagcctccaggcgctctcagtcccgctcctgcgccctcctggagccgcagaggcggctcctcagcggcgctagggggagccccgggtccggagcgggggagcggcggcagccggaccgggagcccctcaacacctgcccctgtggcagagccgcgacaagccaggcggcagctccgagcggggagggcaagtgac

SEQ ID NO: 18466 - RNA, 3348 nt, Homo sapiens
  source 1..3348: mol_type = other RNA
tgagctgctgtaccaaaataccacaaactgcatggcttaaaacaacagaaatttattccctcacaatcctggaggccagatgtctgaaatcaagatattggtagggttggttccttctcgagactctgagggagaatctgtgacatgcctgttttcctagcttctagtgacttcctccaattcttagggttctttggctcatagatgcattgctctaatctctgcctccatcttcccatggccttcagctctgtgtgtctatttccccttcttttctaagagctagtcattgaatttagggcccaccctactacaggttgatctcatttccaggtccttgatttcatctgcaaaaactttttccaaataatgtcacacgtggagattcccagtgaatgtatctcctgggggccactattcagcctattacactattcttagaagatgcctagaaggatatggccaatgttatccagaaggcttcatgaaggaggtaatagaagctaacccttcaaagatgaaagttggcgttcattagagggtcacaaggggaggaagggaatgtcaggttcagggaccagccagaccagagctaaggaagtgacatcacatggaacaatttgtgaacagcaagcagtagggcctggctgcaggacagggtgtgaagtgggggagcagtgatcaggagggccagagagatcagcagggatgtgatcttgagaagctgtgtgtgccatgatctggccctattaatccagaagggtctgatggaagcctctgtgattctcttccatggttaaacattttaattgtattatacctcggatattcctaaatatttaaaacactggcatggttgaactagacaacctttaagtagtttgttccaaccatgagatttagatttcatgatttaggttttatgatcttaaactgaaacctgttagttttctaccactagtgagatcatggcctctgcttttctcctgggaagtccctcttataatcactctcttcccatgattaaagggctactctgccttcatgttgctacccgctcccctggaaatggagaatcaagcaaggatgcggttttccttccattactacatccatacaagagtaaatcaagaataaaagtccagttaatgaaaagatcactggtcttaatatacttagcaaaattttaaaggcaattaaaagtatatacatagacaatgatcaaaattctaatgaaaagacccggctctcccctaaaagaagaaaaaatcatgtaatgtatatatgcattccataaaaacatacatggggaaaacttcagaagcctaaaaacaaaacatcagtaaaccaagccacacttagaaaaatgaaagctgatttttattttatcatcaacagccattctttagacatgaacatgcatacgtaatattctacgcacacatcacagcttttaacgttagttaataaaggttaaacacacaacatacatccttacaaaaaaagtcaaaatgcaaacttaaaactttaaacaaaagtattactaatttaaaaaaagtttgtgttgggtaccatttgtacaacacagttaatttaaacattttcattttggttgcacatgaaaaaggcggcagtagaaaataaagtcattgagggtttttaaatagcagaataggcagttttgccatgcaggagaagcaatattaaatattagtttcaaaaaaaatccacatttaaaaatatttagttcaagtcacagaatttttctcagtagagaccccaatgcaatgcataattagctgccttagatggcccgtttgaaaggatgatatcccttcagagtgtaactttactgattttggcacagaaaagaagtcttaagaacatgattaaaaaagagggaagaggaacagaggaaagaaataaaagcaagaataaatgagatagtaattgcaatcactaaaaaactgcattctcagtcattgcagaatactgtcttctgtctacagcaggtgcttattccagaattgttattgcagcatggatttaatttgcttggaggtagtctcatcattcaaatgttttgttgtgtacctgagagcatttagaagaccttccacactattaggaggttggtccttaagaactttgatacaacctttcatatcaattttggaagttttagcaaatgctcccactggatgtacgtggtcatagagtattatgacacccaccattaccctcaagcagaatgacactgtctcttcatttgtaaatctgcttctgtattccggtgtttccagcatgactctgcatacactagccattgtgcttaaacaatctgtggtattttctattggtaaatttttattctctgatacaaattttgttgtggcatcactcaaggttttcagcattggagttgcctcagcataaaacaaagacattcgatttgccaattcattatttacttcattttctccttctgccggtacattgttaatcctcatacgactcaatgttcttctataatagctgaaatcattctgtatggcaggatttgtcatcttgagttcatcaaaccggagtgtgaaatgaagaatttctgcaaactgtttagcaagagcctgctctcgctctagatgctgggtgggagaatatggggtacttgttaaggctcccagaagacctcttaatgctgcttctaacctctgagaaaattcgtaaaatttctttaatttgcctactagtggaacaactgcaccccatgccttctcttgcaacttctcatctgctggatgctggattgcctctcgtatttcgtggccagctcctctgtatgactgcaagtcctccaagatgccttctgcatcttttaatactacattcacctgattataaatttccttctcagactctgtaggctgggcatcttcagccagtgctggtgattctgtccttgtccttctatccttggattggcgttccctctttcctagttcacttgttccagtccttcaacttctgtttcttgctaacaggtgtgcaaatgaattacctgagaagtgcaaggttggttcagaatacctactgttttcaccacccaactgggtaaccttgaatgagttaatcaaattccaggcctcagtttcttctcctggcggcccgggcgggcgaggggagcgcggcgcgggagcgcaggagcctcggagcctccggtgccgccgccgccgccgtttccgggttggcggggctcacgtcaccgccacaggtttgcgagctgcccccgccgcggcggcagcagcagcagcagcagcagcccgggcgagtgccaggcgagaaataact

SEQ ID NO: 18467 - RNA, 3248 nt, Homo sapiens
  source 1..3248: mol_type = other RNA
tgagctgctgtaccaaaataccacaaactgcatggcttaaaacaacagaaatttattccctcacaatcctggaggccagatgtctgaaatcaagatattggtagggttggttccttctcgagactctgagggagaatctgtgacatgcctgttttcctagcttctagtgacttcctccaattcttagggttctttggctcatagatgcattgctctaatctctgcctccatcttcccatggccttcagctctgtgtgtctatttccccttcttttctaagagctagtcattgaatttagggcccaccctactacaggttgatctcatttccaggtccttgatttcatctgcaaaaactttttccaaataatgtcacacgtggagattcccagtgaatgtatctcctgggggccactattcagcctattacactattcttagaagatgcctagaaggatatggccaatgttatccagaaggcttcatgaaggaggtaatagaagctaacccttcaaagatgaaagttggcgttcattagagggtcacaaggggaggaagggaatgtcaggttcagggaccagccagaccagagctaaggaagtgacatcacatggaacaatttgtgaacagcaagcagtagggcctggctgcaggacagggtgtgaagtgggggagcagtgatcaggagggccagagagatcagcagggatgtgatcttgagaagctgtgtgtgccatgatctggccctattaatccagaagggtctgatggaagcctctgtgattctcttccatggttaaacattttaattgtattatacctcggatattcctaaatatttaaaacactggcatggttgaactagacaacctttaagtagtttgttccaaccatgagatttagatttcatgatttaggttttatgatcttaaactgaaacctgttagttttctaccactagtgagatcatggcctctgcttttctcctgggaagtccctcttataatcactctcttcccatgattaaagggctactctgccttcatgttgctacccgctcccctggaaatggagaatcaagcaaggatgcggttttccttccattactacatccatacaagagtaaatcaagaataaaagtccagttaatgaaaagatcactggtcttaatatacttagcaaaattttaaaggcaattaaaagtatatacatagacaatgatcaaaattctaatgaaaagacccggctctcccctaaaagaagaaaaaatcatgtaatgtatatatgcattccataaaaacatacatggggaaaacttcagaagcctaaaaacaaaacatcagtaaaccaagccacacttagaaaaatgaaagctgatttttattttatcatcaacagccattctttagacatgaacatgcatacgtaatattctacgcacacatcacagcttttaacgttagttaataaaggttaaacacacaacatacatccttacaaaaaaagtcaaaatgcaaacttaaaactttaaacaaaagtattactaatttaaaaaaagtttgtgttgggtaccatttgtacaacacagttaatttaaacattttcattttggttgcacatgaaaaaggcggcagtagaaaataaagtcattgagggtttttaaatagcagaataggcagttttgccatgcaggagaagcaatattaaatattagtttcaaaaaaaatccacatttaaaaatatttagttcaagtcacagaatttttctcagtagagaccccaatgcaatgcataattagctgccttagatggcccgtttgaaaggatgatatcccttcagagtgtaactttactgattttggcacagaaaagaagtcttaagaacatgattaaaaaagagggaagaggaacagaggaaagaaataaaagcaagaataaatgagatagtaattgcaatcactaaaaaactgcattctcagtcattgcagaatactgtcttctgtctacagcaggtgcttattccagaattgttattgcagcatggatttaatttgcttggaggtagtctcatcattcaaatgttttgttgtgtacctgagagcatttagaagaccttccacactattaggaggttggtccttaagaactttgatacaacctttcatatcaattttggaagttttagcaaatgctcccactggatgtacgtggtcatagagtattatgacacccaccattaccctcaagcagaatgacactgtctcttcatttgtaaatctgcttctgtattccggtgtttccagcatgactctgcatacactagccattgtgcttaaacaatctgtggtattttctattggtaaatttttattctctgatacaaattttgttgtggcatcactcaaggttttcagcattggagttgcctcagcataaaacaaagacattcgatttgccaattcattatttacttcattttctccttctgccggtacattgttaatcctcatacgactcaatgttcttctataatagctgaaatcattctgtatggcaggatttgtcatcttgagttcatcaaaccggagtgtgaaatgaagaatttctgcaaactgtttagcaagagcctgctctcgctctagatgctgggtgggagaatatggggtacttgttaaggctcccagaagacctcttaatgctgcttctaacctctgagaaaattcgtaaaatttctttaatttgcctactagtggaacaactgcaccccatgccttctcttgcaacttctcatctgctggatgctggattgcctctcgtatttcgtggccagctcctctgtatgactgcaagtcctccaagatgccttctgcatcttttaatactacattcacctgattataaatttccttctcagactctgtaggctgggcatcttcagccagtgctggtgattctgtccttgtccttctatccttggattggcgttccctctttcctagttcacttgttccagtccttcaacttctgtttcttgctaacaggtgtgcaaatgaattacctgagaagtgcaaggttggttcagaatacctactgttttcaccacccaactgggtaaccttgaatgagttaatcaaattccaggcctcagtttcttctccttcgagaagccgagccgccggcgctcgcacaaaaggaggacgctcgcctcgcgacgcgcctccccccgcgcccagtccccgccgcatcgc

SEQ ID NO: 18468 - RNA, 3249 nt, Homo sapiens
  source 1..3249: mol_type = other RNA
tgagctgctgtaccaaaataccacaaactgcatggcttaaaacaacagaaatttattccctcacaatcctggaggccagatgtctgaaatcaagatattggtagggttggttccttctcgagactctgagggagaatctgtgacatgcctgttttcctagcttctagtgacttcctccaattcttagggttctttggctcatagatgcattgctctaatctctgcctccatcttcccatggccttcagctctgtgtgtctatttccccttcttttctaagagctagtcattgaatttagggcccaccctactacaggttgatctcatttccaggtccttgatttcatctgcaaaaactttttccaaataatgtcacacgtggagattcccagtgaatgtatctcctgggggccactattcagcctattacactattcttagaagatgcctagaaggatatggccaatgttatccagaaggcttcatgaaggaggtaatagaagctaacccttcaaagatgaaagttggcgttcattagagggtcacaaggggaggaagggaatgtcaggttcagggaccagccagaccagagctaaggaagtgacatcacatggaacaatttgtgaacagcaagcagtagggcctggctgcaggacagggtgtgaagtgggggagcagtgatcaggagggccagagagatcagcagggatgtgatcttgagaagctgtgtgtgccatgatctggccctattaatccagaagggtctgatggaagcctctgtgattctcttccatggttaaacattttaattgtattatacctcggatattcctaaatatttaaaacactggcatggttgaactagacaacctttaagtagtttgttccaaccatgagatttagatttcatgatttaggttttatgatcttaaactgaaacctgttagttttctaccactagtgagatcatggcctctgcttttctcctgggaagtccctcttataatcactctcttcccatgattaaagggctactctgccttcatgttgctacccgctcccctggaaatggagaatcaagcaaggatgcggttttccttccattactacatccatacaagagtaaatcaagaataaaagtccagttaatgaaaagatcactggtcttaatatacttagcaaaattttaaaggcaattaaaagtatatacatagacaatgatcaaaattctaatgaaaagacccggctctcccctaaaagaagaaaaaatcatgtaatgtatatatgcattccataaaaacatacatggggaaaacttcagaagcctaaaaacaaaacatcagtaaaccaagccacacttagaaaaatgaaagctgatttttattttatcatcaacagccattctttagacatgaacatgcatacgtaatattctacgcacacatcacagcttttaacgttagttaataaaggttaaacacacaacatacatccttacaaaaaaagtcaaaatgcaaacttaaaactttaaacaaaagtattactaatttaaaaaaagtttgtgttgggtaccatttgtacaacacagttaatttaaacattttcattttggttgcacatgaaaaaggcggcagtagaaaataaagtcattgagggtttttaaatagcagaataggcagttttgccatgcaggagaagcaatattaaatattagtttcaaaaaaaatccacatttaaaaatatttagttcaagtcacagaatttttctcagtagagaccccaatgcaatgcataattagctgccttagatggcccgtttgaaaggatgatatcccttcagagtgtaactttactgattttggcacagaaaagaagtcttaagaacatgattaaaaaagagggaagaggaacagaggaaagaaataaaagcaagaataaatgagatagtaattgcaatcactaaaaaactgcattctcagtcattgcagaatactgtcttctgtctacagcaggtgcttattccagaattgttattgcagcatggatttaatttgcttggaggtagtctcatcattcaaatgttttgttgtgtacctgagagcatttagaagaccttccacactattaggaggttggtccttaagaactttgatacaacctttcatatcaattttggaagttttagcaaatgctcccactggatgtacgtggtcatagagtattatgacacccaccattaccctcaagcagaatgacactgtctcttcatttgtaaatctgcttctgtattccggtgtttccagcatgactctgcatacactagccattgtgcttaaacaatctgtggtattttctattggtaaatttttattctctgatacaaattttgttgtggcatcactcaaggttttcagcattggagttgcctcagcataaaacaaagacattcgatttgccaattcattatttacttcattttctccttctgccggtacattgttaatcctcatacgactcaatgttcttctataatagctgaaatcattctgtatggcaggatttgtcatcttgagttcatcaaaccggagtgtgaaatgaagaatttctgcaaactgtttagcaagagcctgctctcgctctagatgctgggtgggagaatatggggtacttgttaaggctcccagaagacctcttaatgctgcttctaacctctgagaaaattcgtaaaatttctttaatttgcctactagtggaacaactgcaccccatgccttctcttgcaacttctcatctgctggatgctggattgcctctcgtatttcgtggccagctcctctgtatgactgcaagtcctccaagatgccttctgcatcttttaatactacattcacctgattataaatttccttctcagactctgtaggctgggcatcttcagccagtgctggtgattctgtccttgtccttctatccttggattggcgttccctctttcctagttcacttgttccagtccttcaacttctgtttcttgctaacaggtgtgcaaatgaattacctggcggcccgggcgggcgaggggagcgcggcgcgggagcgcaggagcctcggagcctccggtgccgccgccgccgccgtttccgggttggcggggctcacgtcaccgccacaggtttgcgagctgcccccgccgcggcggcagcagcagcagcagcagcagcccgggcgagtgccaggcgagaaataact

SEQ ID NO: 18469 - RNA, 3149 nt, Homo sapiens
  source 1..3149: mol_type = other RNA
tgagctgctgtaccaaaataccacaaactgcatggcttaaaacaacagaaatttattccctcacaatcctggaggccagatgtctgaaatcaagatattggtagggttggttccttctcgagactctgagggagaatctgtgacatgcctgttttcctagcttctagtgacttcctccaattcttagggttctttggctcatagatgcattgctctaatctctgcctccatcttcccatggccttcagctctgtgtgtctatttccccttcttttctaagagctagtcattgaatttagggcccaccctactacaggttgatctcatttccaggtccttgatttcatctgcaaaaactttttccaaataatgtcacacgtggagattcccagtgaatgtatctcctgggggccactattcagcctattacactattcttagaagatgcctagaaggatatggccaatgttatccagaaggcttcatgaaggaggtaatagaagctaacccttcaaagatgaaagttggcgttcattagagggtcacaaggggaggaagggaatgtcaggttcagggaccagccagaccagagctaaggaagtgacatcacatggaacaatttgtgaacagcaagcagtagggcctggctgcaggacagggtgtgaagtgggggagcagtgatcaggagggccagagagatcagcagggatgtgatcttgagaagctgtgtgtgccatgatctggccctattaatccagaagggtctgatggaagcctctgtgattctcttccatggttaaacattttaattgtattatacctcggatattcctaaatatttaaaacactggcatggttgaactagacaacctttaagtagtttgttccaaccatgagatttagatttcatgatttaggttttatgatcttaaactgaaacctgttagttttctaccactagtgagatcatggcctctgcttttctcctgggaagtccctcttataatcactctcttcccatgattaaagggctactctgccttcatgttgctacccgctcccctggaaatggagaatcaagcaaggatgcggttttccttccattactacatccatacaagagtaaatcaagaataaaagtccagttaatgaaaagatcactggtcttaatatacttagcaaaattttaaaggcaattaaaagtatatacatagacaatgatcaaaattctaatgaaaagacccggctctcccctaaaagaagaaaaaatcatgtaatgtatatatgcattccataaaaacatacatggggaaaacttcagaagcctaaaaacaaaacatcagtaaaccaagccacacttagaaaaatgaaagctgatttttattttatcatcaacagccattctttagacatgaacatgcatacgtaatattctacgcacacatcacagcttttaacgttagttaataaaggttaaacacacaacatacatccttacaaaaaaagtcaaaatgcaaacttaaaactttaaacaaaagtattactaatttaaaaaaagtttgtgttgggtaccatttgtacaacacagttaatttaaacattttcattttggttgcacatgaaaaaggcggcagtagaaaataaagtcattgagggtttttaaatagcagaataggcagttttgccatgcaggagaagcaatattaaatattagtttcaaaaaaaatccacatttaaaaatatttagttcaagtcacagaatttttctcagtagagaccccaatgcaatgcataattagctgccttagatggcccgtttgaaaggatgatatcccttcagagtgtaactttactgattttggcacagaaaagaagtcttaagaacatgattaaaaaagagggaagaggaacagaggaaagaaataaaagcaagaataaatgagatagtaattgcaatcactaaaaaactgcattctcagtcattgcagaatactgtcttctgtctacagcaggtgcttattccagaattgttattgcagcatggatttaatttgcttggaggtagtctcatcattcaaatgttttgttgtgtacctgagagcatttagaagaccttccacactattaggaggttggtccttaagaactttgatacaacctttcatatcaattttggaagttttagcaaatgctcccactggatgtacgtggtcatagagtattatgacacccaccattaccctcaagcagaatgacactgtctcttcatttgtaaatctgcttctgtattccggtgtttccagcatgactctgcatacactagccattgtgcttaaacaatctgtggtattttctattggtaaatttttattctctgatacaaattttgttgtggcatcactcaaggttttcagcattggagttgcctcagcataaaacaaagacattcgatttgccaattcattatttacttcattttctccttctgccggtacattgttaatcctcatacgactcaatgttcttctataatagctgaaatcattctgtatggcaggatttgtcatcttgagttcatcaaaccggagtgtgaaatgaagaatttctgcaaactgtttagcaagagcctgctctcgctctagatgctgggtgggagaatatggggtacttgttaaggctcccagaagacctcttaatgctgcttctaacctctgagaaaattcgtaaaatttctttaatttgcctactagtggaacaactgcaccccatgccttctcttgcaacttctcatctgctggatgctggattgcctctcgtatttcgtggccagctcctctgtatgactgcaagtcctccaagatgccttctgcatcttttaatactacattcacctgattataaatttccttctcagactctgtaggctgggcatcttcagccagtgctggtgattctgtccttgtccttctatccttggattggcgttccctctttcctagttcacttgttccagtccttcaacttctgtttcttgctaacaggtgtgcaaatgaattaccttcgagaagccgagccgccggcgctcgcacaaaaggaggacgctcgcctcgcgacgcgcctccccccgcgcccagtccccgccgcatcgc

SEQ ID NO: 18470 - RNA, 3261 nt, Homo sapiens
  source 1..3261: mol_type = other RNA
tgagctgctgtaccaaaataccacaaactgcatggcttaaaacaacagaaatttattccctcacaatcctggaggccagatgtctgaaatcaagatattggtagggttggttccttctcgagactctgagggagaatctgtgacatgcctgttttcctagcttctagtgacttcctccaattcttagggttctttggctcatagatgcattgctctaatctctgcctccatcttcccatggccttcagctctgtgtgtctatttccccttcttttctaagagctagtcattgaatttagggcccaccctactacaggttgatctcatttccaggtccttgatttcatctgcaaaaactttttccaaataatgtcacacgtggagattcccagtgaatgtatctcctgggggccactattcagcctattacactattcttagaagatgcctagaaggatatggccaatgttatccagaaggcttcatgaaggaggtaatagaagctaacccttcaaagatgaaagttggcgttcattagagggtcacaaggggaggaagggaatgtcaggttcagggaccagccagaccagagctaaggaagtgacatcacatggaacaatttgtgaacagcaagcagtagggcctggctgcaggacagggtgtgaagtgggggagcagtgatcaggagggccagagagatcagcagggatgtgatcttgagaagctgtgtgtgccatgatctggccctattaatccagaagggtctgatggaagcctctgtgattctcttccatggttaaacattttaattgtattatacctcggatattcctaaatatttaaaacactggcatggttgaactagacaacctttaagtagtttgttccaaccatgagatttagatttcatgatttaggttttatgatcttaaactgaaacctgttagttttctaccactagtgagatcatggcctctgcttttctcctgggaagtccctcttataatcactctcttcccatgattaaagggctactctgccttcatgttgctacccgctcccctggaaatggagaatcaagcaaggatgcggttttccttccattactacatccatacaagagtaaatcaagaataaaagtccagttaatgaaaagatcactggtcttaatatacttagcaaaattttaaaggcaattaaaagtatatacatagacaatgatcaaaattctaatgaaaagacccggctctcccctaaaagaagaaaaaatcatgtaatgtatatatgcattccataaaaacatacatggggaaaacttcagaagcctaaaaacaaaacatcagtaaaccaagccacacttagaaaaatgaaagctgatttttattttatcatcaacagccattctttagacatgaacatgcatacgtaatattctacgcacacatcacagcttttaacgttagttaataaaggttaaacacacaacatacatccttacaaaaaaagtcaaaatgcaaacttaaaactttaaacaaaagtattactaatttaaaaaaagtttgtgttgggtaccatttgtacaacacagttaatttaaacattttcattttggttgcacatgaaaaaggcggcagtagaaaataaagtcattgagggtttttaaatagcagaataggcagttttgccatgcaggagaagcaatattaaatattagtttcaaaaaaaatccacatttaaaaatatttagttcaagtcacagaatttttctcagtagagaccccaatgcaatgcataattagctgccttagatggcccgtttgaaaggatgatatcccttcagagtgtaactttactgattttggcacagaaaagaagtcttaagaacatgattaaaaaagagggaagaggaacagaggaaagaaataaaagcaagaataaatgagatagtaattgcaatcactaaaaaactgcattctcagtcattgcagaatactgtcttctgtctacagcaggtgcttattccagaattgttattgcagcatggatttaatttgcttggaggtagtctcatcattcaaatgttttgttgtgtacctgagagcatttagaagaccttccacactattaggaggttggtccttaagaactttgatacaacctttcatatcaattttggaagttttagcaaatgctcccactggatgtacgtggtcatagagtattatgacacccaccattaccctcaagcagaatgacactgtctcttcatttgtaaatctgcttctgtattccggtgtttccagcatgactctgcatacactagccattgtgcttaaacaatctgtggtattttctattggtaaatttttattctctgatacaaattttgttgtggcatcactcaaggttttcagcattggagttgcctcagcataaaacaaagacattcgatttgccaattcattatttacttcattttctccttctgccggtacattgttaatcctcatacgactcaatgttcttctataatagctgaaatcattctgtatggcaggatttgtcatcttgagttcatcaaaccggagtgtgaaatgaagaatttctgcaaactgtttagcaagagcctgctctcgctctagatgctgggtgggagaatatggggtacttgttaaggctcccagaagacctcttaatgctgcttctaacctctgagaaaattcgtaaaatttctttaatttgcctactagtggaacaactgcaccccatgccttctcttgcaacttctcatctgctggatgctggattgcctctcgtatttcgtggccagctcctctgtatgactgcaagtcctccaagatgccttctgcatcttttaatactacattcacctgattataaatttccttctcagactctgtaggctgggcatcttcagccagtgctggtgattctgtccttgtccttctatctgagaagtgcaaggttggttcagaatacctactgttttcaccacccaactgggtaaccttgaatgagttaatcaaattccaggcctcagtttcttctcctggcggcccgggcgggcgaggggagcgcggcgcgggagcgcaggagcctcggagcctccggtgccgccgccgccgccgtttccgggttggcggggctcacgtcaccgccacaggtttgcgagctgcccccgccgcggcggcagcagcagcagcagcagcagcccgggcgagtgccaggcgagaaataact

SEQ ID NO: 18471 - RNA, 3162 nt, Homo sapiens
  source 1..3162: mol_type = other RNA
tgagctgctgtaccaaaataccacaaactgcatggcttaaaacaacagaaatttattccctcacaatcctggaggccagatgtctgaaatcaagatattggtagggttggttccttctcgagactctgagggagaatctgtgacatgcctgttttcctagcttctagtgacttcctccaattcttagggttctttggctcatagatgcattgctctaatctctgcctccatcttcccatggccttcagctctgtgtgtctatttccccttcttttctaagagctagtcattgaatttagggcccaccctactacaggttgatctcatttccaggtccttgatttcatctgcaaaaactttttccaaataatgtcacacgtggagattcccagtgaatgtatctcctgggggccactattcagcctattacactattcttagaagatgcctagaaggatatggccaatgttatccagaaggcttcatgaaggaggtaatagaagctaacccttcaaagatgaaagttggcgttcattagagggtcacaaggggaggaagggaatgtcaggttcagggaccagccagaccagagctaaggaagtgacatcacatggaacaatttgtgaacagcaagcagtagggcctggctgcaggacagggtgtgaagtgggggagcagtgatcaggagggccagagagatcagcagggatgtgatcttgagaagctgtgtgtgccatgatctggccctattaatccagaagggtctgatggaagcctctgtgattctcttccatggttaaacattttaattgtattatacctcggatattcctaaatatttaaaacactggcatggttgaactagacaacctttaagtagtttgttccaaccatgagatttagatttcatgatttaggttttatgatcttaaactgaaacctgttagttttctaccactagtgagatcatggcctctgcttttctcctgggaagtccctcttataatcactctcttcccatgattaaagggctactctgccttcatgttgctacccgctcccctggaaatggagaatcaagcaaggatgcggttttccttccattactacatccatacaagagtaaatcaagaataaaagtccagttaatgaaaagatcactggtcttaatatacttagcaaaattttaaaggcaattaaaagtatatacatagacaatgatcaaaattctaatgaaaagacccggctctcccctaaaagaagaaaaaatcatgtaatgtatatatgcattccataaaaacatacatggggaaaacttcagaagcctaaaaacaaaacatcagtaaaccaagccacacttagaaaaatgaaagctgatttttattttatcatcaacagccattctttagacatgaacatgcatacgtaatattctacgcacacatcacagcttttaacgttagttaataaaggttaaacacacaacatacatccttacaaaaaaagtcaaaatgcaaacttaaaactttaaacaaaagtattactaatttaaaaaaagtttgtgttgggtaccatttgtacaacacagttaatttaaacattttcattttggttgcacatgaaaaaggcggcagtagaaaataaagtcattgagggtttttaaatagcagaataggcagttttgccatgcaggagaagcaatattaaatattagtttcaaaaaaaatccacatttaaaaatatttagttcaagtcacagaatttttctcagtagagaccccaatgcaatgcataattagctgccttagatggcccgtttgaaaggatgatatcccttcagagtgtaactttactgattttggcacagaaaagaagtcttaagaacatgattaaaaaagagggaagaggaacagaggaaagaaataaaagcaagaataaatgagatagtaattgcaatcactaaaaaactgcattctcagtcattgcagaatactgtcttctgtctacagcaggtgcttattccagaattgttattgcagcatggatttaatttgcttggaggtagtctcatcattcaaatgttttgttgtgtacctgagagcatttagaagaccttccacactattaggaggttggtccttaagaactttgatacaacctttcatatcaattttggaagttttagcaaatgctcccactggatgtacgtggtcatagagtattatgacacccaccattaccctcaagcagaatgacactgtctcttcatttgtaaatctgcttctgtattccggtgtttccagcatgactctgcatacactagccattgtgcttaaacaatctgtggtattttctattggtaaatttttattctctgatacaaattttgttgtggcatcactcaaggttttcagcattggagttgcctcagcataaaacaaagacattcgatttgccaattcattatttacttcattttctccttctgccggtacattgttaatcctcatacgactcaatgttcttctataatagctgaaatcattctgtatggcaggatttgtcatcttgagttcatcaaaccggagtgtgaaatgaagaatttctgcaaactgtttagcaagagcctgctctcgctctagatgctgggtgggagaatatggggtacttgttaaggctcccagaagacctcttaatgctgcttctaacctctgagaaaattcgtaaaatttctttaatttgcctactagtggaacaactgcaccccatgccttctcttgcaacttctcatctgctggatgctggattgcctctcgtatttcgtggccagctcctctgtatgactgcaagtcctccaagatgccttctgcatcttttaatactacattcacctgattataaatttccttctcagactctgtaggctgggcatcttcagccagtgctggtgattctgtccttgtccttctatctggcggcccgggcgggcgaggggagcgcggcgcgggagcgcaggagcctcggagcctccggtgccgccgccgccgccgtttccgggttggcggggctcacgtcaccgccacaggtttgcgagctgcccccgccgcggcggcagcagcagcagcagcagcagcccgggcgagtgccaggcgagaaataact

SEQ ID NO: 18472 - RNA, 3246 nt, Homo sapiens
  source 1..3246: mol_type = other RNA
tgagctgctgtaccaaaataccacaaactgcatggcttaaaacaacagaaatttattccctcacaatcctggaggccagatgtctgaaatcaagatattggtagggttggttccttctcgagactctgagggagaatctgtgacatgcctgttttcctagcttctagtgacttcctccaattcttagggttctttggctcatagatgcattgctctaatctctgcctccatcttcccatggccttcagctctgtgtgtctatttccccttcttttctaagagctagtcattgaatttagggcccaccctactacaggttgatctcatttccaggtccttgatttcatctgcaaaaactttttccaaataatgtcacacgtggagattcccagtgaatgtatctcctgggggccactattcagcctattacactattcttagaagatgcctagaaggatatggccaatgttatccagaaggcttcatgaaggaggtaatagaagctaacccttcaaagatgaaagttggcgttcattagagggtcacaaggggaggaagggaatgtcaggttcagggaccagccagaccagagctaaggaagtgacatcacatggaacaatttgtgaacagcaagcagtagggcctggctgcaggacagggtgtgaagtgggggagcagtgatcaggagggccagagagatcagcagggatgtgatcttgagaagctgtgtgtgccatgatctggccctattaatccagaagggtctgatggaagcctctgtgattctcttccatggttaaacattttaattgtattatacctcggatattcctaaatatttaaaacactggcatggttgaactagacaacctttaagtagtttgttccaaccatgagatttagatttcatgatttaggttttatgatcttaaactgaaacctgttagttttctaccactagtgagatcatggcctctgcttttctcctgggaagtccctcttataatcactctcttcccatgattaaagggctactctgccttcatgttgctacccgctcccctggaaatggagaatcaagcaaggatgcggttttccttccattactacatccatacaagagtaaatcaagaataaaagtccagttaatgaaaagatcactggtcttaatatacttagcaaaattttaaaggcaattaaaagtatatacatagacaatgatcaaaattctaatgaaaagacccggctctcccctaaaagaagaaaaaatcatgtaatgtatatatgcattccataaaaacatacatggggaaaacttcagaagcctaaaaacaaaacatcagtaaaccaagccacacttagaaaaatgaaagctgatttttattttatcatcaacagccattctttagacatgaacatgcatacgtaatattctacgcacacatcacagcttttaacgttagttaataaaggttaaacacacaacatacatccttacaaaaaaagtcaaaatgcaaacttaaaactttaaacaaaagtattactaatttaaaaaaagtttgtgttgggtaccatttgtacaacacagttaatttaaacattttcattttggttgcacatgaaaaaggcggcagtagaaaataaagtcattgagggtttttaaatagcagaataggcagttttgccatgcaggagaagcaatattaaatattagtttcaaaaaaaatccacatttaaaaatatttagttcaagtcacagaatttttctcagtagagaccccaatgcaatgcataattagctgccttagatggcccgtttgaaaggatgatatcccttcagagtgtaactttactgattttggcacagaaaagaagtcttaagaacatgattaaaaaagagggaagaggaacagaggaaagaaataaaagcaagaataaatgagatagtaattgcaatcactaaaaaactgcattctcagtcattgcagaatactgtcttctgtctacagcaggtgcttattccagaattgttattgcagcatggatttaatttgcttggaggtagtctcatcattcaaatgttttgttgtgtacctgagagcatttagaagaccttccacactattaggaggttggtccttaagaactttgatacaacctttcatatcaattttggaagttttagcaaatgctcccactggatgtacgtggtcatagagtattatgacacccaccattaccctcaagcagaatgacactgtctcttcatttgtaaatctgcttctgtattccggtgtttccagcatgactctgcatacactagccattgtgcttaaacaatctgtggtattttctattggtaaatttttattctctgatacaaattttgttgtggcatcactcaaggttttcagcattggagttgcctcagcataaaacaaagacattcgatttgccaattcattatttacttcattttctccttctgccggtacattgttaatcctcatacgactcaatgttcttctataatagctgaaatcattctgtatggcaggatttgtcatcttgagttcatcaaaccggagtgtgaaatgaagaatttctgcaaactgtttagcaagagcctgctctcgctctagatgctgggtgggagaatatggggtacttgttaaggctcccagaagacctcttaatgctgcttctaacctctgagaaaattcgtaaaatttctttaatttgcctactagtggaacaactgcaccccatgccttctcttgcaacttctcatctgctggatgctggattgcctctcgtatttcgtggccagctcctctgtatgactgcaagtcctccaagatgccttctgcatcttttaatactacattcacctgattataaatttccttctcagactctgtaggctgggcatcttcagccagtgctggtgattctgtccttgtccttctatctgtttaaggaaagaaaaaaaggaagaaagtcaactgggtaaccttgaatgagttaatcaaattccaggcctcagtttcttctcctggcggcccgggcgggcgaggggagcgcggcgcgggagcgcaggagcctcggagcctccggtgccgccgccgccgccgtttccgggttggcggggctcacgtcaccgccacaggtttgcgagctgcccccgccgcggcggcagcagcagcagcagcagcagcccgggcgagtgccaggcgagaaataact

SEQ ID NO: 18473 - RNA, 3321 nt, Homo sapiens
  source 1..3321: mol_type = other RNA
tgagctgctgtaccaaaataccacaaactgcatggcttaaaacaacagaaatttattccctcacaatcctggaggccagatgtctgaaatcaagatattggtagggttggttccttctcgagactctgagggagaatctgtgacatgcctgttttcctagcttctagtgacttcctccaattcttagggttctttggctcatagatgcattgctctaatctctgcctccatcttcccatggccttcagctctgtgtgtctatttccccttcttttctaagagctagtcattgaatttagggcccaccctactacaggttgatctcatttccaggtccttgatttcatctgcaaaaactttttccaaataatgtcacacgtggagattcccagtgaatgtatctcctgggggccactattcagcctattacactattcttagaagatgcctagaaggatatggccaatgttatccagaaggcttcatgaaggaggtaatagaagctaacccttcaaagatgaaagttggcgttcattagagggtcacaaggggaggaagggaatgtcaggttcagggaccagccagaccagagctaaggaagtgacatcacatggaacaatttgtgaacagcaagcagtagggcctggctgcaggacagggtgtgaagtgggggagcagtgatcaggagggccagagagatcagcagggatgtgatcttgagaagctgtgtgtgccatgatctggccctattaatccagaagggtctgatggaagcctctgtgattctcttccatggttaaacattttaattgtattatacctcggatattcctaaatatttaaaacactggcatggttgaactagacaacctttaagtagtttgttccaaccatgagatttagatttcatgatttaggttttatgatcttaaactgaaacctgttagttttctaccactagtgagatcatggcctctgcttttctcctgggaagtccctcttataatcactctcttcccatgattaaagggctactctgccttcatgttgctacccgctcccctggaaatggagaatcaagcaaggatgcggttttccttccattactacatccatacaagagtaaatcaagaataaaagtccagttaatgaaaagatcactggtcttaatatacttagcaaaattttaaaggcaattaaaagtatatacatagacaatgatcaaaattctaatgaaaagacccggctctcccctaaaagaagaaaaaatcatgtaatgtatatatgcattccataaaaacatacatggggaaaacttcagaagcctaaaaacaaaacatcagtaaaccaagccacacttagaaaaatgaaagctgatttttattttatcatcaacagccattctttagacatgaacatgcatacgtaatattctacgcacacatcacagcttttaacgttagttaataaaggttaaacacacaacatacatccttacaaaaaaagtcaaaatgcaaacttaaaactttaaacaaaagtattactaatttaaaaaaagtttgtgttgggtaccatttgtacaacacagttaatttaaacattttcattttggttgcacatgaaaaaggcggcagtagaaaataaagtcattgagggtttttaaatagcagaataggcagttttgccatgcaggagaagcaatattaaatattagtttcaaaaaaaatccacatttaaaaatatttagttcaagtcacagaatttttctcagtagagaccccaatgcaatgcataattagctgccttagatggcccgtttgaaaggatgatatcccttcagagtgtaactttactgattttggcacagaaaagaagtcttaagaacatgattaaaaaagagggaagaggaacagaggaaagaaataaaagcaagaataaatgagatagtaattgcaatcactaaaaaactgcattctcagtcattgcagaatactgtcttctgtctacagcaggtgcttattccagaattgttattgcagcatggatttaatttgcttggaggtagtctcatcattcaaatgttttgttgtgtacctgagagcatttagaagaccttccacactattaggaggttggtccttaagaactttgatacaacctttcatatcaattttggaagttttagcaaatgctcccactggatgtacgtggtcatagagtattatgacacccaccattaccctcaagcagaatgacactgtctcttcatttgtaaatctgcttctgtattccggtgtttccagcatgactctgcatacactagccattgtgcttaaacaatctgtggtattttctattggtaaatttttattctctgatacaaattttgttgtggcatcactcaaggttttcagcattggagttgcctcagcataaaacaaagacattcgatttgccaattcattatttacttcattttctccttctgccggtacattgttaatcctcatacgactcaatgttcttctataatagctgaaatcattctgtatggcaggatttgtcatcttgagttcatcaaaccggagtgtgaaatgaagaatttctgcaaactgtttagcaagagcctgctctcgctctagatgctgggtgggagaatatggggtacttgttaaggctcccagaagacctcttaatgctgcttctaacctctgagaaaattcgtaaaatttctttaatttgcctactagtggaacaactgcaccccatgccttctcttgcaacttctcatctgctggatgctggattgcctctcgtatttcgtggccagctcctctgtatgactgcaagtcctccaagatgccttctgcatcttttaatactacattcacctgattataaatttccttctcagactctgtaggctgggcattgccaagtaaacaggccttgtggcagtgaaaggataaactgtccatcattctttcttctcctcggagatttcacaggaaaaggagaaagcgcaggaaacaggaggccttcagccagtgctggtgattctgtccttgtccttctatcaactgggtaaccttgaatgagttaatcaaattccaggcctcagtttcttctcctggcggcccgggcgggcgaggggagcgcggcgcgggagcgcaggagcctcggagcctccggtgccgccgccgccgccgtttccgggttggcggggctcacgtcaccgccacaggtttgcgagctgcccccgccgcggcggcagcagcagcagcagcagcagcccgggcgagtgccaggcgagaaataact

SEQ ID NO: 18474 - RNA, 3259 nt, Homo sapiens
  source 1..3259: mol_type = other RNA
tgagctgctgtaccaaaataccacaaactgcatggcttaaaacaacagaaatttattccctcacaatcctggaggccagatgtctgaaatcaagatattggtagggttggttccttctcgagactctgagggagaatctgtgacatgcctgttttcctagcttctagtgacttcctccaattcttagggttctttggctcatagatgcattgctctaatctctgcctccatcttcccatggccttcagctctgtgtgtctatttccccttcttttctaagagctagtcattgaatttagggcccaccctactacaggttgatctcatttccaggtccttgatttcatctgcaaaaactttttccaaataatgtcacacgtggagattcccagtgaatgtatctcctgggggccactattcagcctattacactattcttagaagatgcctagaaggatatggccaatgttatccagaaggcttcatgaaggaggtaatagaagctaacccttcaaagatgaaagttggcgttcattagagggtcacaaggggaggaagggaatgtcaggttcagggaccagccagaccagagctaaggaagtgacatcacatggaacaatttgtgaacagcaagcagtagggcctggctgcaggacagggtgtgaagtgggggagcagtgatcaggagggccagagagatcagcagggatgtgatcttgagaagctgtgtgtgccatgatctggccctattaatccagaagggtctgatggaagcctctgtgattctcttccatggttaaacattttaattgtattatacctcggatattcctaaatatttaaaacactggcatggttgaactagacaacctttaagtagtttgttccaaccatgagatttagatttcatgatttaggttttatgatcttaaactgaaacctgttagttttctaccactagtgagatcatggcctctgcttttctcctgggaagtccctcttataatcactctcttcccatgattaaagggctactctgccttcatgttgctacccgctcccctggaaatggagaatcaagcaaggatgcggttttccttccattactacatccatacaagagtaaatcaagaataaaagtccagttaatgaaaagatcactggtcttaatatacttagcaaaattttaaaggcaattaaaagtatatacatagacaatgatcaaaattctaatgaaaagacccggctctcccctaaaagaagaaaaaatcatgtaatgtatatatgcattccataaaaacatacatggggaaaacttcagaagcctaaaaacaaaacatcagtaaaccaagccacacttagaaaaatgaaagctgatttttattttatcatcaacagccattctttagacatgaacatgcatacgtaatattctacgcacacatcacagcttttaacgttagttaataaaggttaaacacacaacatacatccttacaaaaaaagtcaaaatgcaaacttaaaactttaaacaaaagtattactaatttaaaaaaagtttgtgttgggtaccatttgtacaacacagttaatttaaacattttcattttggttgcacatgaaaaaggcggcagtagaaaataaagtcattgagggtttttaaatagcagaataggcagttttgccatgcaggagaagcaatattaaatattagtttcaaaaaaaatccacatttaaaaatatttagttcaagtcacagaatttttctcagtagagaccccaatgcaatgcataattagctgccttagatggcccgtttgaaaggatgatatcccttcagagtgtaactttactgattttggcacagaaaagaagtcttaagaacatgattaaaaaagagggaagaggaacagaggaaagaaataaaagcaagaataaatgagatagtaattgcaatcactaaaaaactgcattctcagtcattgcagaatactgtcttctgtctacagcaggtgcttattccagaattgttattgcagcatggatttaatttgcttggaggtagtctcatcattcaaatgttttgttgtgtacctgagagcatttagaagaccttccacactattaggaggttggtccttaagaactttgatacaacctttcatatcaattttggaagttttagcaaatgctcccactggatgtacgtggtcatagagtattatgacacccaccattaccctcaagcagaatgacactgtctcttcatttgtaaatctgcttctgtattccggtgtttccagcatgactctgcatacactagccattgtgcttaaacaatctgtggtattttctattggtaaatttttattctctgatacaaattttgttgtggcatcactcaaggttttcagcattggagttgcctcagcataaaacaaagacattcgatttgccaattcattatttacttcattttctccttctgccggtacattgttaatcctcatacgactcaatgttcttctataatagctgaaatcattctgtatggcaggatttgtcatcttgagttcatcaaaccggagtgtgaaatgaagaatttctgcaaactgtttagcaagagcctgctctcgctctagatgctgggtgggagaatatggggtacttgttaaggctcccagaagacctcttaatgctgcttctaacctctgagaaaattcgtaaaatttctttaatttgcctactagtggaacaactgcaccccatgccttctcttgcaacttctcatctgctggatgctggattgcctctcgtatttcgtggccagctcctctgtatgactgcaagtcctccaagatgccttctgcatcttttaatactacattcacctgattataaatttccttctcagactctgtaggctgggcattttcaaaatcaaggaaaaaatttggcccctgctcaaggtctgtgcatgtcaaaactttaagaagattccccatgttaaggtaccaactgggtaaccttgaatgagttaatcaaattccaggcctcagtttcttctcctggcggcccgggcgggcgaggggagcgcggcgcgggagcgcaggagcctcggagcctccggtgccgccgccgccgccgtttccgggttggcggggctcacgtcaccgccacaggtttgcgagctgcccccgccgcggcggcagcagcagcagcagcagcagcccgggcgagtgccaggcgagaaataact

SEQ ID NO: 18475 - RNA, 3219 nt, Homo sapiens
  source 1..3219: mol_type = other RNA
tgagctgctgtaccaaaataccacaaactgcatggcttaaaacaacagaaatttattccctcacaatcctggaggccagatgtctgaaatcaagatattggtagggttggttccttctcgagactctgagggagaatctgtgacatgcctgttttcctagcttctagtgacttcctccaattcttagggttctttggctcatagatgcattgctctaatctctgcctccatcttcccatggccttcagctctgtgtgtctatttccccttcttttctaagagctagtcattgaatttagggcccaccctactacaggttgatctcatttccaggtccttgatttcatctgcaaaaactttttccaaataatgtcacacgtggagattcccagtgaatgtatctcctgggggccactattcagcctattacactattcttagaagatgcctagaaggatatggccaatgttatccagaaggcttcatgaaggaggtaatagaagctaacccttcaaagatgaaagttggcgttcattagagggtcacaaggggaggaagggaatgtcaggttcagggaccagccagaccagagctaaggaagtgacatcacatggaacaatttgtgaacagcaagcagtagggcctggctgcaggacagggtgtgaagtgggggagcagtgatcaggagggccagagagatcagcagggatgtgatcttgagaagctgtgtgtgccatgatctggccctattaatccagaagggtctgatggaagcctctgtgattctcttccatggttaaacattttaattgtattatacctcggatattcctaaatatttaaaacactggcatggttgaactagacaacctttaagtagtttgttccaaccatgagatttagatttcatgatttaggttttatgatcttaaactgaaacctgttagttttctaccactagtgagatcatggcctctgcttttctcctgggaagtccctcttataatcactctcttcccatgattaaagggctactctgccttcatgttgctacccgctcccctggaaatggagaatcaagcaaggatgcggttttccttccattactacatccatacaagagtaaatcaagaataaaagtccagttaatgaaaagatcactggtcttaatatacttagcaaaattttaaaggcaattaaaagtatatacatagacaatgatcaaaattctaatgaaaagacccggctctcccctaaaagaagaaaaaatcatgtaatgtatatatgcattccataaaaacatacatggggaaaacttcagaagcctaaaaacaaaacatcagtaaaccaagccacacttagaaaaatgaaagctgatttttattttatcatcaacagccattctttagacatgaacatgcatacgtaatattctacgcacacatcacagcttttaacgttagttaataaaggttaaacacacaacatacatccttacaaaaaaagtcaaaatgcaaacttaaaactttaaacaaaagtattactaatttaaaaaaagtttgtgttgggtaccatttgtacaacacagttaatttaaacattttcattttggttgcacatgaaaaaggcggcagtagaaaataaagtcattgagggtttttaaatagcagaataggcagttttgccatgcaggagaagcaatattaaatattagtttcaaaaaaaatccacatttaaaaatatttagttcaagtcacagaatttttctcagtagagaccccaatgcaatgcataattagctgccttagatggcccgtttgaaaggatgatatcccttcagagtgtaactttactgattttggcacagaaaagaagtcttaagaacatgattaaaaaagagggaagaggaacagaggaaagaaataaaagcaagaataaatgagatagtaattgcaatcactaaaaaactgcattctcagtcattgcagaatactgtcttctgtctacagcaggtgcttattccagaattgttattgcagcatggatttaatttgcttggaggtagtctcatcattcaaatgttttgttgtgtacctgagagcatttagaagaccttccacactattaggaggttggtccttaagaactttgatacaacctttcatatcaattttggaagttttagcaaatgctcccactggatgtacgtggtcatagagtattatgacacccaccattaccctcaagcagaatgacactgtctcttcatttgtaaatctgcttctgtattccggtgtttccagcatgactctgcatacactagccattgtgcttaaacaatctgtggtattttctattggtaaatttttattctctgatacaaattttgttgtggcatcactcaaggttttcagcattggagttgcctcagcataaaacaaagacattcgatttgccaattcattatttacttcattttctccttctgccggtacattgttaatcctcatacgactcaatgttcttctataatagctgaaatcattctgtatggcaggatttgtcatcttgagttcatcaaaccggagtgtgaaatgaagaatttctgcaaactgtttagcaagagcctgctctcgctctagatgctgggtgggagaatatggggtacttgttaaggctcccagaagacctcttaatgctgcttctaacctctgagaaaattcgtaaaatttctttaatttgcctactagtggaacaactgcaccccatgccttctcttgcaacttctcatctgctggatgctggattgcctctcgtatttcgtggccagctcctctgtatgactgcaagtcctccaagatgccttctgcatcttttaatactacattcacctgattataaatttccttctcagactctgtaggctgggcattttcaaaatcaaggaaaaaatttggcccctgctcaaggtctgtgcatgtcaaaactttaagaagattccccatgttaaggtaccctccgctcgagcctccaggcgctctcagtcccgctcctgcgccctcctggagccgcagaggcggctcctcagcggcgctagggggagccccgggtccggagcgggggagcggcggcagccggaccgggagcccctcaacacctgcccctgtggcagagccgcgacaagccaggcggcagctccgagcggggagggcaagtgac

SEQ ID NO: 18476 - RNA, 3481 nt, Homo sapiens
  source 1..3481: mol_type = other RNA
tgagctgctgtaccaaaataccacaaactgcatggcttaaaacaacagaaatttattccctcacaatcctggaggccagatgtctgaaatcaagatattggtagggttggttccttctcgagactctgagggagaatctgtgacatgcctgttttcctagcttctagtgacttcctccaattcttagggttctttggctcatagatgcattgctctaatctctgcctccatcttcccatggccttcagctctgtgtgtctatttccccttcttttctaagagctagtcattgaatttagggcccaccctactacaggttgatctcatttccaggtccttgatttcatctgcaaaaactttttccaaataatgtcacacgtggagattcccagtgaatgtatctcctgggggccactattcagcctattacactattcttagaagatgcctagaaggatatggccaatgttatccagaaggcttcatgaaggaggtaatagaagctaacccttcaaagatgaaagttggcgttcattagagggtcacaaggggaggaagggaatgtcaggttcagggaccagccagaccagagctaaggaagtgacatcacatggaacaatttgtgaacagcaagcagtagggcctggctgcaggacagggtgtgaagtgggggagcagtgatcaggagggccagagagatcagcagggatgtgatcttgagaagctgtgtgtgccatgatctggccctattaatccagaagggtctgatggaagcctctgtgattctcttccatggttaaacattttaattgtattatacctcggatattcctaaatatttaaaacactggcatggttgaactagacaacctttaagtagtttgttccaaccatgagatttagatttcatgatttaggttttatgatcttaaactgaaacctgttagttttctaccactagtgagatcatggcctctgcttttctcctgggaagtccctcttataatcactctcttcccatgattaaagggctactctgccttcatgttgctacccgctcccctggaaatggagaatcaagcaaggatgcggttttccttccattactacatccatacaagagtaaatcaagaataaaagtccagttaatgaaaagatcactggtcttaatatacttagcaaaattttaaaggcaattaaaagtatatacatagacaatgatcaaaattctaatgaaaagacccggctctcccctaaaagaagaaaaaatcatgtaatgtatatatgcattccataaaaacatacatggggaaaacttcagaagcctaaaaacaaaacatcagtaaaccaagccacacttagaaaaatgaaagctgatttttattttatcatcaacagccattctttagacatgaacatgcatacgtaatattctacgcacacatcacagcttttaacgttagttaataaaggttaaacacacaacatacatccttacaaaaaaagtcaaaatgcaaacttaaaactttaaacaaaagtattactaatttaaaaaaagtttgtgttgggtaccatttgtacaacacagttaatttaaacattttcattttggttgcacatgaaaaaggcggcagtagaaaataaagtcattgagggtttttaaatagcagaataggcagttttgccatgcaggagaagcaatattaaatattagtttcaaaaaaaatccacatttaaaaatatttagttcaagtcacagaatttttctcagtagagaccccaatgcaatgcataattagctgccttagatggcccgtttgaaaggatgatatcccttcagagtgtaactttactgattttggcacagaaaagaagtcttaagaacatgattaaaaaagagggaagaggaacagaggaaagaaataaaagcaagaataaatgagatagtaattgcaatcactaaaaaactgcattctcagtcattgcagaatactgtcttctgtctacagcaggtgcttattccagaattgttattgcagcatggatttaatttgcttggaggtagtctcatcattcaaatgttttgttgtgtacctgagagcatttagaagaccttccacactattaggaggttggtccttaagaactttgatacaacctttcatatcaattttggaagttttagcaaatgctcccactggatgtacgtggtcatagagtattatgacacccaccattaccctcaagcagaatgacactgtctcttcatttgtaaatctgcttctgtattccggtgtttccagcatgactctgcatacactagccattgtgcttaaacaatctgtggtattttctattggtaaatttttattctctgatacaaattttgttgtggcatcactcaaggttttcagcattggagttgcctcagcataaaacaaagacattcgatttgccaattcattatttacttcattttctccttctgccggtacattgttaatcctcatacgactcaatgttcttctataatagctgaaatcattctgtatggcaggatttgtcatcttgagttcatcaaaccggagtgtgaaatgaagaatttctgcaaactgtttagcaagagcctgctctcgctctagatgctgggtgggagaatatggggtacttgttaaggctcccagaagacctcttaatgctgcttctaacctctgagaaaattcgtaaaatttctttaatttgcctactagtggaacaactgcaccccatgccttctcttgcaacttctcatctgctggatgctggattgcctctcgtatttcgtggccagctcctctgtatgactgcaagtcctccaagatgccttctgcatcttttaatactacattcacctgattataaatttccttctcagactctgtaggctgggcattttcaaaatcaaggaaaaaatttggcccctgctcaaggtctgtgcatgtcaaaactttaagaagattccccatgttaaggtacctccccagagtgagagtctctggtgcctcttccagtcaccaaacagcagcaaaaaagcaaggaacttaaggacctactgccaagtaaacaggccttgtggcagtgaaaggataaactgtccatcattctttcttctcctcggagatttcacaggaaaaggagaaagcgcaggaaacaggaggccttcagccagtgctggtgattctgtccttgtccttctatcaactgggtaaccttgaatgagttaatcaaattccaggcctcagtttcttctcctggcggcccgggcgggcgaggggagcgcggcgcgggagcgcaggagcctcggagcctccggtgccgccgccgccgccgtttccgggttggcggggctcacgtcaccgccacaggtttgcgagctgcccccgccgcggcggcagcagcagcagcagcagcagcccgggcgagtgccaggcgagaaataact

SEQ ID NO: 18477 - RNA, 3381 nt, Homo sapiens
  source 1..3381: mol_type = other RNA
tgagctgctgtaccaaaataccacaaactgcatggcttaaaacaacagaaatttattccctcacaatcctggaggccagatgtctgaaatcaagatattggtagggttggttccttctcgagactctgagggagaatctgtgacatgcctgttttcctagcttctagtgacttcctccaattcttagggttctttggctcatagatgcattgctctaatctctgcctccatcttcccatggccttcagctctgtgtgtctatttccccttcttttctaagagctagtcattgaatttagggcccaccctactacaggttgatctcatttccaggtccttgatttcatctgcaaaaactttttccaaataatgtcacacgtggagattcccagtgaatgtatctcctgggggccactattcagcctattacactattcttagaagatgcctagaaggatatggccaatgttatccagaaggcttcatgaaggaggtaatagaagctaacccttcaaagatgaaagttggcgttcattagagggtcacaaggggaggaagggaatgtcaggttcagggaccagccagaccagagctaaggaagtgacatcacatggaacaatttgtgaacagcaagcagtagggcctggctgcaggacagggtgtgaagtgggggagcagtgatcaggagggccagagagatcagcagggatgtgatcttgagaagctgtgtgtgccatgatctggccctattaatccagaagggtctgatggaagcctctgtgattctcttccatggttaaacattttaattgtattatacctcggatattcctaaatatttaaaacactggcatggttgaactagacaacctttaagtagtttgttccaaccatgagatttagatttcatgatttaggttttatgatcttaaactgaaacctgttagttttctaccactagtgagatcatggcctctgcttttctcctgggaagtccctcttataatcactctcttcccatgattaaagggctactctgccttcatgttgctacccgctcccctggaaatggagaatcaagcaaggatgcggttttccttccattactacatccatacaagagtaaatcaagaataaaagtccagttaatgaaaagatcactggtcttaatatacttagcaaaattttaaaggcaattaaaagtatatacatagacaatgatcaaaattctaatgaaaagacccggctctcccctaaaagaagaaaaaatcatgtaatgtatatatgcattccataaaaacatacatggggaaaacttcagaagcctaaaaacaaaacatcagtaaaccaagccacacttagaaaaatgaaagctgatttttattttatcatcaacagccattctttagacatgaacatgcatacgtaatattctacgcacacatcacagcttttaacgttagttaataaaggttaaacacacaacatacatccttacaaaaaaagtcaaaatgcaaacttaaaactttaaacaaaagtattactaatttaaaaaaagtttgtgttgggtaccatttgtacaacacagttaatttaaacattttcattttggttgcacatgaaaaaggcggcagtagaaaataaagtcattgagggtttttaaatagcagaataggcagttttgccatgcaggagaagcaatattaaatattagtttcaaaaaaaatccacatttaaaaatatttagttcaagtcacagaatttttctcagtagagaccccaatgcaatgcataattagctgccttagatggcccgtttgaaaggatgatatcccttcagagtgtaactttactgattttggcacagaaaagaagtcttaagaacatgattaaaaaagagggaagaggaacagaggaaagaaataaaagcaagaataaatgagatagtaattgcaatcactaaaaaactgcattctcagtcattgcagaatactgtcttctgtctacagcaggtgcttattccagaattgttattgcagcatggatttaatttgcttggaggtagtctcatcattcaaatgttttgttgtgtacctgagagcatttagaagaccttccacactattaggaggttggtccttaagaactttgatacaacctttcatatcaattttggaagttttagcaaatgctcccactggatgtacgtggtcatagagtattatgacacccaccattaccctcaagcagaatgacactgtctcttcatttgtaaatctgcttctgtattccggtgtttccagcatgactctgcatacactagccattgtgcttaaacaatctgtggtattttctattggtaaatttttattctctgatacaaattttgttgtggcatcactcaaggttttcagcattggagttgcctcagcataaaacaaagacattcgatttgccaattcattatttacttcattttctccttctgccggtacattgttaatcctcatacgactcaatgttcttctataatagctgaaatcattctgtatggcaggatttgtcatcttgagttcatcaaaccggagtgtgaaatgaagaatttctgcaaactgtttagcaagagcctgctctcgctctagatgctgggtgggagaatatggggtacttgttaaggctcccagaagacctcttaatgctgcttctaacctctgagaaaattcgtaaaatttctttaatttgcctactagtggaacaactgcaccccatgccttctcttgcaacttctcatctgctggatgctggattgcctctcgtatttcgtggccagctcctctgtatgactgcaagtcctccaagatgccttctgcatcttttaatactacattcacctgattataaatttccttctcagactctgtaggctgggcattttcaaaatcaaggaaaaaatttggcccctgctcaaggtctgtgcatgtcaaaactttaagaagattccccatgttaaggtacctccccagagtgagagtctctggtgcctcttccagtcaccaaacagcagcaaaaaagcaaggaacttaaggacctactgccaagtaaacaggccttgtggcagtgaaaggataaactgtccatcattctttcttctcctcggagatttcacaggaaaaggagaaagcgcaggaaacaggaggccttcagccagtgctggtgattctgtccttgtccttctatcaactgggtaaccttgaatgagttaatcaaattccaggcctcagtttcttctccttcgagaagccgagccgccggcgctcgcacaaaaggaggacgctcgcctcgcgacgcgcctccccccgcgcccagtccccgccgcatcgc

SEQ ID NO: 18478 - RNA, 3441 nt, Homo sapiens
  source 1..3441: mol_type = other RNA
tgagctgctgtaccaaaataccacaaactgcatggcttaaaacaacagaaatttattccctcacaatcctggaggccagatgtctgaaatcaagatattggtagggttggttccttctcgagactctgagggagaatctgtgacatgcctgttttcctagcttctagtgacttcctccaattcttagggttctttggctcatagatgcattgctctaatctctgcctccatcttcccatggccttcagctctgtgtgtctatttccccttcttttctaagagctagtcattgaatttagggcccaccctactacaggttgatctcatttccaggtccttgatttcatctgcaaaaactttttccaaataatgtcacacgtggagattcccagtgaatgtatctcctgggggccactattcagcctattacactattcttagaagatgcctagaaggatatggccaatgttatccagaaggcttcatgaaggaggtaatagaagctaacccttcaaagatgaaagttggcgttcattagagggtcacaaggggaggaagggaatgtcaggttcagggaccagccagaccagagctaaggaagtgacatcacatggaacaatttgtgaacagcaagcagtagggcctggctgcaggacagggtgtgaagtgggggagcagtgatcaggagggccagagagatcagcagggatgtgatcttgagaagctgtgtgtgccatgatctggccctattaatccagaagggtctgatggaagcctctgtgattctcttccatggttaaacattttaattgtattatacctcggatattcctaaatatttaaaacactggcatggttgaactagacaacctttaagtagtttgttccaaccatgagatttagatttcatgatttaggttttatgatcttaaactgaaacctgttagttttctaccactagtgagatcatggcctctgcttttctcctgggaagtccctcttataatcactctcttcccatgattaaagggctactctgccttcatgttgctacccgctcccctggaaatggagaatcaagcaaggatgcggttttccttccattactacatccatacaagagtaaatcaagaataaaagtccagttaatgaaaagatcactggtcttaatatacttagcaaaattttaaaggcaattaaaagtatatacatagacaatgatcaaaattctaatgaaaagacccggctctcccctaaaagaagaaaaaatcatgtaatgtatatatgcattccataaaaacatacatggggaaaacttcagaagcctaaaaacaaaacatcagtaaaccaagccacacttagaaaaatgaaagctgatttttattttatcatcaacagccattctttagacatgaacatgcatacgtaatattctacgcacacatcacagcttttaacgttagttaataaaggttaaacacacaacatacatccttacaaaaaaagtcaaaatgcaaacttaaaactttaaacaaaagtattactaatttaaaaaaagtttgtgttgggtaccatttgtacaacacagttaatttaaacattttcattttggttgcacatgaaaaaggcggcagtagaaaataaagtcattgagggtttttaaatagcagaataggcagttttgccatgcaggagaagcaatattaaatattagtttcaaaaaaaatccacatttaaaaatatttagttcaagtcacagaatttttctcagtagagaccccaatgcaatgcataattagctgccttagatggcccgtttgaaaggatgatatcccttcagagtgtaactttactgattttggcacagaaaagaagtcttaagaacatgattaaaaaagagggaagaggaacagaggaaagaaataaaagcaagaataaatgagatagtaattgcaatcactaaaaaactgcattctcagtcattgcagaatactgtcttctgtctacagcaggtgcttattccagaattgttattgcagcatggatttaatttgcttggaggtagtctcatcattcaaatgttttgttgtgtacctgagagcatttagaagaccttccacactattaggaggttggtccttaagaactttgatacaacctttcatatcaattttggaagttttagcaaatgctcccactggatgtacgtggtcatagagtattatgacacccaccattaccctcaagcagaatgacactgtctcttcatttgtaaatctgcttctgtattccggtgtttccagcatgactctgcatacactagccattgtgcttaaacaatctgtggtattttctattggtaaatttttattctctgatacaaattttgttgtggcatcactcaaggttttcagcattggagttgcctcagcataaaacaaagacattcgatttgccaattcattatttacttcattttctccttctgccggtacattgttaatcctcatacgactcaatgttcttctataatagctgaaatcattctgtatggcaggatttgtcatcttgagttcatcaaaccggagtgtgaaatgaagaatttctgcaaactgtttagcaagagcctgctctcgctctagatgctgggtgggagaatatggggtacttgttaaggctcccagaagacctcttaatgctgcttctaacctctgagaaaattcgtaaaatttctttaatttgcctactagtggaacaactgcaccccatgccttctcttgcaacttctcatctgctggatgctggattgcctctcgtatttcgtggccagctcctctgtatgactgcaagtcctccaagatgccttctgcatcttttaatactacattcacctgattataaatttccttctcagactctgtaggctgggcattttcaaaatcaaggaaaaaatttggcccctgctcaaggtctgtgcatgtcaaaactttaagaagattccccatgttaaggtacctccccagagtgagagtctctggtgcctcttccagtcaccaaacagcagcaaaaaagcaaggaacttaaggacctactgccaagtaaacaggccttgtggcagtgaaaggataaactgtccatcattctttcttctcctcggagatttcacaggaaaaggagaaagcgcaggaaacaggaggccttcagccagtgctggtgattctgtccttgtccttctatcctccgctcgagcctccaggcgctctcagtcccgctcctgcgccctcctggagccgcagaggcggctcctcagcggcgctagggggagccccgggtccggagcgggggagcggcggcagccggaccgggagcccctcaacacctgcccctgtggcagagccgcgacaagccaggcggcagctccgagcggggagggcaagtgac

SEQ ID NO: 18479 - RNA, 3568 nt, Homo sapiens
  source 1..3568: mol_type = other RNA
tgagctgctgtaccaaaataccacaaactgcatggcttaaaacaacagaaatttattccctcacaatcctggaggccagatgtctgaaatcaagatattggtagggttggttccttctcgagactctgagggagaatctgtgacatgcctgttttcctagcttctagtgacttcctccaattcttagggttctttggctcatagatgcattgctctaatctctgcctccatcttcccatggccttcagctctgtgtgtctatttccccttcttttctaagagctagtcattgaatttagggcccaccctactacaggttgatctcatttccaggtccttgatttcatctgcaaaaactttttccaaataatgtcacacgtggagattcccagtgaatgtatctcctgggggccactattcagcctattacactattcttagaagatgcctagaaggatatggccaatgttatccagaaggcttcatgaaggaggtaatagaagctaacccttcaaagatgaaagttggcgttcattagagggtcacaaggggaggaagggaatgtcaggttcagggaccagccagaccagagctaaggaagtgacatcacatggaacaatttgtgaacagcaagcagtagggcctggctgcaggacagggtgtgaagtgggggagcagtgatcaggagggccagagagatcagcagggatgtgatcttgagaagctgtgtgtgccatgatctggccctattaatccagaagggtctgatggaagcctctgtgattctcttccatggttaaacattttaattgtattatacctcggatattcctaaatatttaaaacactggcatggttgaactagacaacctttaagtagtttgttccaaccatgagatttagatttcatgatttaggttttatgatcttaaactgaaacctgttagttttctaccactagtgagatcatggcctctgcttttctcctgggaagtccctcttataatcactctcttcccatgattaaagggctactctgccttcatgttgctacccgctcccctggaaatggagaatcaagcaaggatgcggttttccttccattactacatccatacaagagtaaatcaagaataaaagtccagttaatgaaaagatcactggtcttaatatacttagcaaaattttaaaggcaattaaaagtatatacatagacaatgatcaaaattctaatgaaaagacccggctctcccctaaaagaagaaaaaatcatgtaatgtatatatgcattccataaaaacatacatggggaaaacttcagaagcctaaaaacaaaacatcagtaaaccaagccacacttagaaaaatgaaagctgatttttattttatcatcaacagccattctttagacatgaacatgcatacgtaatattctacgcacacatcacagcttttaacgttagttaataaaggttaaacacacaacatacatccttacaaaaaaagtcaaaatgcaaacttaaaactttaaacaaaagtattactaatttaaaaaaagtttgtgttgggtaccatttgtacaacacagttaatttaaacattttcattttggttgcacatgaaaaaggcggcagtagaaaataaagtcattgagggtttttaaatagcagaataggcagttttgccatgcaggagaagcaatattaaatattagtttcaaaaaaaatccacatttaaaaatatttagttcaagtcacagaatttttctcagtagagaccccaatgcaatgcataattagctgccttagatggcccgtttgaaaggatgatatcccttcagagtgtaactttactgattttggcacagaaaagaagtcttaagaacatgattaaaaaagagggaagaggaacagaggaaagaaataaaagcaagaataaatgagatagtaattgcaatcactaaaaaactgcattctcagtcattgcagaatactgtcttctgtctacagcaggtgcttattccagaattgttattgcagcatggatttaatttgcttggaggtagtctcatcattcaaatgttttgttgtgtacctgagagcatttagaagaccttccacactattaggaggttggtccttaagaactttgatacaacctttcatatcaattttggaagttttagcaaatgctcccactggatgtacgtggtcatagagtattatgacacccaccattaccctcaagcagaatgacactgtctcttcatttgtaaatctgcttctgtattccggtgtttccagcatgactctgcatacactagccattgtgcttaaacaatctgtggtattttctattggtaaatttttattctctgatacaaattttgttgtggcatcactcaaggttttcagcattggagttgcctcagcataaaacaaagacattcgatttgccaattcattatttacttcattttctccttctgccggtacattgttaatcctcatacgactcaatgttcttctataatagctgaaatcattctgtatggcaggatttgtcatcttgagttcatcaaaccggagtgtgaaatgaagaatttctgcaaactgtttagcaagagcctgctctcgctctagatgctgggtgggagaatatggggtacttgttaaggctcccagaagacctcttaatgctgcttctaacctctgagaaaattcgtaaaatttctttaatttgcctactagtggaacaactgcaccccatgccttctcttgcaacttctcatctgctggatgctggattgcctctcgtatttcgtggccagctcctctgtatgactgcaagtcctccaagatgccttctgcatcttttaatactacattcacctgattataaatttccttctcagactctgtaggctgggcattttcaaaatcaaggaaaaaatttggcccctgctcaaggtctgtgcatgtcaaaactttaagaagattccccatgttaaggtacctccccagagtgagagtctctggtgcctcttccagtcaccaaacagcagcaaaaaagcaaggaacttaaggacctactgccaagtaaacaggccttgtggcagtgaaaggataaactgtccatcattctttcttctcctcggagatttcacaggaaaaggagaaagcgcaggaaacaggaggccttcagccagtgctggtgattctgtccttgtccttctatccttggattggcgttccctctttcctagttcacttgttccagtccttcaacttctgtttcttgctaacaggtgtgcaaatgaattaccaactgggtaaccttgaatgagttaatcaaattccaggcctcagtttcttctcctggcggcccgggcgggcgaggggagcgcggcgcgggagcgcaggagcctcggagcctccggtgccgccgccgccgccgtttccgggttggcggggctcacgtcaccgccacaggtttgcgagctgcccccgccgcggcggcagcagcagcagcagcagcagcccgggcgagtgccaggcgagaaataact

SEQ ID NO: 18480 - RNA, 3514 nt, Homo sapiens
  source 1..3514: mol_type = other RNA
tgagctgctgtaccaaaataccacaaactgcatggcttaaaacaacagaaatttattccctcacaatcctggaggccagatgtctgaaatcaagatattggtagggttggttccttctcgagactctgagggagaatctgtgacatgcctgttttcctagcttctagtgacttcctccaattcttagggttctttggctcatagatgcattgctctaatctctgcctccatcttcccatggccttcagctctgtgtgtctatttccccttcttttctaagagctagtcattgaatttagggcccaccctactacaggttgatctcatttccaggtccttgatttcatctgcaaaaactttttccaaataatgtcacacgtggagattcccagtgaatgtatctcctgggggccactattcagcctattacactattcttagaagatgcctagaaggatatggccaatgttatccagaaggcttcatgaaggaggtaatagaagctaacccttcaaagatgaaagttggcgttcattagagggtcacaaggggaggaagggaatgtcaggttcagggaccagccagaccagagctaaggaagtgacatcacatggaacaatttgtgaacagcaagcagtagggcctggctgcaggacagggtgtgaagtgggggagcagtgatcaggagggccagagagatcagcagggatgtgatcttgagaagctgtgtgtgccatgatctggccctattaatccagaagggtctgatggaagcctctgtgattctcttccatggttaaacattttaattgtattatacctcggatattcctaaatatttaaaacactggcatggttgaactagacaacctttaagtagtttgttccaaccatgagatttagatttcatgatttaggttttatgatcttaaactgaaacctgttagttttctaccactagtgagatcatggcctctgcttttctcctgggaagtccctcttataatcactctcttcccatgattaaagggctactctgccttcatgttgctacccgctcccctggaaatggagaatcaagcaaggatgcggttttccttccattactacatccatacaagagtaaatcaagaataaaagtccagttaatgaaaagatcactggtcttaatatacttagcaaaattttaaaggcaattaaaagtatatacatagacaatgatcaaaattctaatgaaaagacccggctctcccctaaaagaagaaaaaatcatgtaatgtatatatgcattccataaaaacatacatggggaaaacttcagaagcctaaaaacaaaacatcagtaaaccaagccacacttagaaaaatgaaagctgatttttattttatcatcaacagccattctttagacatgaacatgcatacgtaatattctacgcacacatcacagcttttaacgttagttaataaaggttaaacacacaacatacatccttacaaaaaaagtcaaaatgcaaacttaaaactttaaacaaaagtattactaatttaaaaaaagtttgtgttgggtaccatttgtacaacacagttaatttaaacattttcattttggttgcacatgaaaaaggcggcagtagaaaataaagtcattgagggtttttaaatagcagaataggcagttttgccatgcaggagaagcaatattaaatattagtttcaaaaaaaatccacatttaaaaatatttagttcaagtcacagaatttttctcagtagagaccccaatgcaatgcataattagctgccttagatggcccgtttgaaaggatgatatcccttcagagtgtaactttactgattttggcacagaaaagaagtcttaagaacatgattaaaaaagagggaagaggaacagaggaaagaaataaaagcaagaataaatgagatagtaattgcaatcactaaaaaactgcattctcagtcattgcagaatactgtcttctgtctacagcaggtgcttattccagaattgttattgcagcatggatttaatttgcttggaggtagtctcatcattcaaatgttttgttgtgtacctgagagcatttagaagaccttccacactattaggaggttggtccttaagaactttgatacaacctttcatatcaattttggaagttttagcaaatgctcccactggatgtacgtggtcatagagtattatgacacccaccattaccctcaagcagaatgacactgtctcttcatttgtaaatctgcttctgtattccggtgtttccagcatgactctgcatacactagccattgtgcttaaacaatctgtggtattttctattggtaaatttttattctctgatacaaattttgttgtggcatcactcaaggttttcagcattggagttgcctcagcataaaacaaagacattcgatttgccaattcattatttacttcattttctccttctgccggtacattgttaatcctcatacgactcaatgttcttctataatagctgaaatcattctgtatggcaggatttgtcatcttgagttcatcaaaccggagtgtgaaatgaagaatttctgcaaactgtttagcaagagcctgctctcgctctagatgctgggtgggagaatatggggtacttgttaaggctcccagaagacctcttaatgctgcttctaacctctgagaaaattcgtaaaatttctttaatttgcctactagtggaacaactgcaccccatgccttctcttgcaacttctcatctgctggatgctggattgcctctcgtatttcgtggccagctcctctgtatgactgcaagtcctccaagatgccttctgcatcttttaatactacattcacctgattataaatttccttctcagactctgtaggctgggcattttcaaaatcaaggaaaaaatttggcccctgctcaaggtctgtgcatgtcaaaactttaagaagattccccatgttaaggtacctccccagagtgagagtctctggtgcctcttccagtcaccaaacagcagcaaaaaagcaaggaacttaaggacctactgccaagtaaacaggccttgtggcagtgaaaggataaactgtccatcattctttcttctcctcggagatttcacaggaaaaggagaaagcgcaggaaacaggaggccttcagccagtgctggtgattctgtccttgtccttctatccttggattggcgttccctctttcctagttcacttgttccagtccttcaacttctgtttcttgctaacaggtgtgcaaatgaattacctgagaagtgcaaggttggttcagaatacctactgttttcaccacccaactgggtaaccttgaatgagttaatcaaattccaggcctcagtttcttctccttcgagaagccgagccgccggcgctcgcacaaaaggaggacgctcgcctcgcgacgcgcctccccccgcgcccagtccccgccgcatcgc

SEQ ID NO: 18481 - RNA, 3364 nt, Homo sapiens
  source 1..3364: mol_type = other RNA
tgagctgctgtaccaaaataccacaaactgcatggcttaaaacaacagaaatttattccctcacaatcctggaggccagatgtctgaaatcaagatattggtagggttggttccttctcgagactctgagggagaatctgtgacatgcctgttttcctagcttctagtgacttcctccaattcttagggttctttggctcatagatgcattgctctaatctctgcctccatcttcccatggccttcagctctgtgtgtctatttccccttcttttctaagagctagtcattgaatttagggcccaccctactacaggttgatctcatttccaggtccttgatttcatctgcaaaaactttttccaaataatgtcacacgtggagattcccagtgaatgtatctcctgggggccactattcagcctattacactattcttagaagatgcctagaaggatatggccaatgttatccagaaggcttcatgaaggaggtaatagaagctaacccttcaaagatgaaagttggcgttcattagagggtcacaaggggaggaagggaatgtcaggttcagggaccagccagaccagagctaaggaagtgacatcacatggaacaatttgtgaacagcaagcagtagggcctggctgcaggacagggtgtgaagtgggggagcagtgatcaggagggccagagagatcagcagggatgtgatcttgagaagctgtgtgtgccatgatctggccctattaatccagaagggtctgatggaagcctctgtgattctcttccatggttaaacattttaattgtattatacctcggatattcctaaatatttaaaacactggcatggttgaactagacaacctttaagtagtttgttccaaccatgagatttagatttcatgatttaggttttatgatcttaaactgaaacctgttagttttctaccactagtgagatcatggcctctgcttttctcctgggaagtccctcttataatcactctcttcccatgattaaagggctactctgccttcatgttgctacccgctcccctggaaatggagaatcaagcaaggatgcggttttccttccattactacatccatacaagagtaaatcaagaataaaagtccagttaatgaaaagatcactggtcttaatatacttagcaaaattttaaaggcaattaaaagtatatacatagacaatgatcaaaattctaatgaaaagacccggctctcccctaaaagaagaaaaaatcatgtaatgtatatatgcattccataaaaacatacatggggaaaacttcagaagcctaaaaacaaaacatcagtaaaccaagccacacttagaaaaatgaaagctgatttttattttatcatcaacagccattctttagacatgaacatgcatacgtaatattctacgcacacatcacagcttttaacgttagttaataaaggttaaacacacaacatacatccttacaaaaaaagtcaaaatgcaaacttaaaactttaaacaaaagtattactaatttaaaaaaagtttgtgttgggtaccatttgtacaacacagttaatttaaacattttcattttggttgcacatgaaaaaggcggcagtagaaaataaagtcattgagggtttttaaatagcagaataggcagttttgccatgcaggagaagcaatattaaatattagtttcaaaaaaaatccacatttaaaaatatttagttcaagtcacagaatttttctcagtagagaccccaatgcaatgcataattagctgccttagatggcccgtttgaaaggatgatatcccttcagagtgtaactttactgattttggcacagaaaagaagtcttaagaacatgattaaaaaagagggaagaggaacagaggaaagaaataaaagcaagaataaatgagatagtaattgcaatcactaaaaaactgcattctcagtcattgcagaatactgtcttctgtctacagcaggtgcttattccagaattgttattgcagcatggatttaatttgcttggaggtagtctcatcattcaaatgttttgttgtgtacctgagagcatttagaagaccttccacactattaggaggttggtccttaagaactttgatacaacctttcatatcaattttggaagttttagcaaatgctcccactggatgtacgtggtcatagagtattatgacacccaccattaccctcaagcagaatgacactgtctcttcatttgtaaatctgcttctgtattccggtgtttccagcatgactctgcatacactagccattgtgcttaaacaatctgtggtattttctattggtaaatttttattctctgatacaaattttgttgtggcatcactcaaggttttcagcattggagttgcctcagcataaaacaaagacattcgatttgccaattcattatttacttcattttctccttctgccggtacattgttaatcctcatacgactcaatgttcttctataatagctgaaatcattctgtatggcaggatttgtcatcttgagttcatcaaaccggagtgtgaaatgaagaatttctgcaaactgtttagcaagagcctgctctcgctctagatgctgggtgggagaatatggggtacttgttaaggctcccagaagacctcttaatgctgcttctaacctctgagaaaattcgtaaaatttctttaatttgcctactagtggaacaactgcaccccatgccttctcttgcaacttctcatctgctggatgctggattgcctctcgtatttcgtggccagctcctctgtatgactgcaagtcctccaagatgccttctgcatcttttaatactacattcacctgattataaatttccttctcagactctgtaggctgggcattttcaaaatcaaggaaaaaatttggcccctgctcaaggtctgtgcatgtcaaaactttaagaagattccccatgttaaggtacctctcctaaagaaagaaagcttcagccagtgctggtgattctgtccttgtccttctatccttggattggcgttccctctttcctagttcacttgttccagtccttcaacttctgtttcttgctaacaggtgtgcaaatgaattaccctccgctcgagcctccaggcgctctcagtcccgctcctgcgccctcctggagccgcagaggcggctcctcagcggcgctagggggagccccgggtccggagcgggggagcggcggcagccggaccgggagcccctcaacacctgcccctgtggcagagccgcgacaagccaggcggcagctccgagcggggagggcaagtgac

SEQ ID NO: 18482 - RNA, 3298 nt, Homo sapiens
  source 1..3298: mol_type = other RNA
tgagctgctgtaccaaaataccacaaactgcatggcttaaaacaacagaaatttattccctcacaatcctggaggccagatgtctgaaatcaagatattggtagggttggttccttctcgagactctgagggagaatctgtgacatgcctgttttcctagcttctagtgacttcctccaattcttagggttctttggctcatagatgcattgctctaatctctgcctccatcttcccatggccttcagctctgtgtgtctatttccccttcttttctaagagctagtcattgaatttagggcccaccctactacaggttgatctcatttccaggtccttgatttcatctgcaaaaactttttccaaataatgtcacacgtggagattcccagtgaatgtatctcctgggggccactattcagcctattacactattcttagaagatgcctagaaggatatggccaatgttatccagaaggcttcatgaaggaggtaatagaagctaacccttcaaagatgaaagttggcgttcattagagggtcacaaggggaggaagggaatgtcaggttcagggaccagccagaccagagctaaggaagtgacatcacatggaacaatttgtgaacagcaagcagtagggcctggctgcaggacagggtgtgaagtgggggagcagtgatcaggagggccagagagatcagcagggatgtgatcttgagaagctgtgtgtgccatgatctggccctattaatccagaagggtctgatggaagcctctgtgattctcttccatggttaaacattttaattgtattatacctcggatattcctaaatatttaaaacactggcatggttgaactagacaacctttaagtagtttgttccaaccatgagatttagatttcatgatttaggttttatgatcttaaactgaaacctgttagttttctaccactagtgagatcatggcctctgcttttctcctgggaagtccctcttataatcactctcttcccatgattaaagggctactctgccttcatgttgctacccgctcccctggaaatggagaatcaagcaaggatgcggttttccttccattactacatccatacaagagtaaatcaagaataaaagtccagttaatgaaaagatcactggtcttaatatacttagcaaaattttaaaggcaattaaaagtatatacatagacaatgatcaaaattctaatgaaaagacccggctctcccctaaaagaagaaaaaatcatgtaatgtatatatgcattccataaaaacatacatggggaaaacttcagaagcctaaaaacaaaacatcagtaaaccaagccacacttagaaaaatgaaagctgatttttattttatcatcaacagccattctttagacatgaacatgcatacgtaatattctacgcacacatcacagcttttaacgttagttaataaaggttaaacacacaacatacatccttacaaaaaaagtcaaaatgcaaacttaaaactttaaacaaaagtattactaatttaaaaaaagtttgtgttgggtaccatttgtacaacacagttaatttaaacattttcattttggttgcacatgaaaaaggcggcagtagaaaataaagtcattgagggtttttaaatagcagaataggcagttttgccatgcaggagaagcaatattaaatattagtttcaaaaaaaatccacatttaaaaatatttagttcaagtcacagaatttttctcagtagagaccccaatgcaatgcataattagctgccttagatggcccgtttgaaaggatgatatcccttcagagtgtaactttactgattttggcacagaaaagaagtcttaagaacatgattaaaaaagagggaagaggaacagaggaaagaaataaaagcaagaataaatgagatagtaattgcaatcactaaaaaactgcattctcagtcattgcagaatactgtcttctgtctacagcaggtgcttattccagaattgttattgcagcatggatttaatttgcttggaggtagtctcatcattcaaatgttttgttgtgtacctgagagcatttagaagaccttccacactattaggaggttggtccttaagaactttgatacaacctttcatatcaattttggaagttttagcaaatgctcccactggatgtacgtggtcatagagtattatgacacccaccattaccctcaagcagaatgacactgtctcttcatttgtaaatctgcttctgtattccggtgtttccagcatgactctgcatacactagccattgtgcttaaacaatctgtggtattttctattggtaaatttttattctctgatacaaattttgttgtggcatcactcaaggttttcagcattggagttgcctcagcataaaacaaagacattcgatttgccaattcattatttacttcattttctccttctgccggtacattgttaatcctcatacgactcaatgttcttctataatagctgaaatcattctgtatggcaggatttgtcatcttgagttcatcaaaccggagtgtgaaatgaagaatttctgcaaactgtttagcaagagcctgctctcgctctagatgctgggtgggagaatatggggtacttgttaaggctcccagaagacctcttaatgctgcttctaacctctgagaaaattcgtaaaatttctttaatttgcctactagtggaacaactgcaccccatgccttctcttgcaacttctcatctgctggatgctggattgcctctcgtatttcgtggccagctcctctgtatgactgcaagtcctccaagatgccttctgcatcttttaatactacattcacctgattataaatttccttctcagactctgtaggctgggcattttcaaaatcaaggaaaaaatttggcccctgctcaaggtctgtgcatgtcaaaactttaagaagattccccatgttaaggtaccttcagccagtgctggtgattctgtccttgtccttctatcaactgggtaaccttgaatgagttaatcaaattccaggcctcagtttcttctcctggcggcccgggcgggcgaggggagcgcggcgcgggagcgcaggagcctcggagcctccggtgccgccgccgccgccgtttccgggttggcggggctcacgtcaccgccacaggtttgcgagctgcccccgccgcggcggcagcagcagcagcagcagcagcccgggcgagtgccaggcgagaaataact

SEQ ID NO: 18483 - RNA, 3198 nt, Homo sapiens
  source 1..3198: mol_type = other RNA
tgagctgctgtaccaaaataccacaaactgcatggcttaaaacaacagaaatttattccctcacaatcctggaggccagatgtctgaaatcaagatattggtagggttggttccttctcgagactctgagggagaatctgtgacatgcctgttttcctagcttctagtgacttcctccaattcttagggttctttggctcatagatgcattgctctaatctctgcctccatcttcccatggccttcagctctgtgtgtctatttccccttcttttctaagagctagtcattgaatttagggcccaccctactacaggttgatctcatttccaggtccttgatttcatctgcaaaaactttttccaaataatgtcacacgtggagattcccagtgaatgtatctcctgggggccactattcagcctattacactattcttagaagatgcctagaaggatatggccaatgttatccagaaggcttcatgaaggaggtaatagaagctaacccttcaaagatgaaagttggcgttcattagagggtcacaaggggaggaagggaatgtcaggttcagggaccagccagaccagagctaaggaagtgacatcacatggaacaatttgtgaacagcaagcagtagggcctggctgcaggacagggtgtgaagtgggggagcagtgatcaggagggccagagagatcagcagggatgtgatcttgagaagctgtgtgtgccatgatctggccctattaatccagaagggtctgatggaagcctctgtgattctcttccatggttaaacattttaattgtattatacctcggatattcctaaatatttaaaacactggcatggttgaactagacaacctttaagtagtttgttccaaccatgagatttagatttcatgatttaggttttatgatcttaaactgaaacctgttagttttctaccactagtgagatcatggcctctgcttttctcctgggaagtccctcttataatcactctcttcccatgattaaagggctactctgccttcatgttgctacccgctcccctggaaatggagaatcaagcaaggatgcggttttccttccattactacatccatacaagagtaaatcaagaataaaagtccagttaatgaaaagatcactggtcttaatatacttagcaaaattttaaaggcaattaaaagtatatacatagacaatgatcaaaattctaatgaaaagacccggctctcccctaaaagaagaaaaaatcatgtaatgtatatatgcattccataaaaacatacatggggaaaacttcagaagcctaaaaacaaaacatcagtaaaccaagccacacttagaaaaatgaaagctgatttttattttatcatcaacagccattctttagacatgaacatgcatacgtaatattctacgcacacatcacagcttttaacgttagttaataaaggttaaacacacaacatacatccttacaaaaaaagtcaaaatgcaaacttaaaactttaaacaaaagtattactaatttaaaaaaagtttgtgttgggtaccatttgtacaacacagttaatttaaacattttcattttggttgcacatgaaaaaggcggcagtagaaaataaagtcattgagggtttttaaatagcagaataggcagttttgccatgcaggagaagcaatattaaatattagtttcaaaaaaaatccacatttaaaaatatttagttcaagtcacagaatttttctcagtagagaccccaatgcaatgcataattagctgccttagatggcccgtttgaaaggatgatatcccttcagagtgtaactttactgattttggcacagaaaagaagtcttaagaacatgattaaaaaagagggaagaggaacagaggaaagaaataaaagcaagaataaatgagatagtaattgcaatcactaaaaaactgcattctcagtcattgcagaatactgtcttctgtctacagcaggtgcttattccagaattgttattgcagcatggatttaatttgcttggaggtagtctcatcattcaaatgttttgttgtgtacctgagagcatttagaagaccttccacactattaggaggttggtccttaagaactttgatacaacctttcatatcaattttggaagttttagcaaatgctcccactggatgtacgtggtcatagagtattatgacacccaccattaccctcaagcagaatgacactgtctcttcatttgtaaatctgcttctgtattccggtgtttccagcatgactctgcatacactagccattgtgcttaaacaatctgtggtattttctattggtaaatttttattctctgatacaaattttgttgtggcatcactcaaggttttcagcattggagttgcctcagcataaaacaaagacattcgatttgccaattcattatttacttcattttctccttctgccggtacattgttaatcctcatacgactcaatgttcttctataatagctgaaatcattctgtatggcaggatttgtcatcttgagttcatcaaaccggagtgtgaaatgaagaatttctgcaaactgtttagcaagagcctgctctcgctctagatgctgggtgggagaatatggggtacttgttaaggctcccagaagacctcttaatgctgcttctaacctctgagaaaattcgtaaaatttctttaatttgcctactagtggaacaactgcaccccatgccttctcttgcaacttctcatctgctggatgctggattgcctctcgtatttcgtggccagctcctctgtatgactgcaagtcctccaagatgccttctgcatcttttaatactacattcacctgattataaatttccttctcagactctgtaggctgggcattttcaaaatcaaggaaaaaatttggcccctgctcaaggtctgtgcatgtcaaaactttaagaagattccccatgttaaggtaccttcagccagtgctggtgattctgtccttgtccttctatcaactgggtaaccttgaatgagttaatcaaattccaggcctcagtttcttctccttcgagaagccgagccgccggcgctcgcacaaaaggaggacgctcgcctcgcgacgcgcctccccccgcgcccagtccccgccgcatcgc

SEQ ID NO: 18484 - RNA, 3258 nt, Homo sapiens
  source 1..3258: mol_type = other RNA
tgagctgctgtaccaaaataccacaaactgcatggcttaaaacaacagaaatttattccctcacaatcctggaggccagatgtctgaaatcaagatattggtagggttggttccttctcgagactctgagggagaatctgtgacatgcctgttttcctagcttctagtgacttcctccaattcttagggttctttggctcatagatgcattgctctaatctctgcctccatcttcccatggccttcagctctgtgtgtctatttccccttcttttctaagagctagtcattgaatttagggcccaccctactacaggttgatctcatttccaggtccttgatttcatctgcaaaaactttttccaaataatgtcacacgtggagattcccagtgaatgtatctcctgggggccactattcagcctattacactattcttagaagatgcctagaaggatatggccaatgttatccagaaggcttcatgaaggaggtaatagaagctaacccttcaaagatgaaagttggcgttcattagagggtcacaaggggaggaagggaatgtcaggttcagggaccagccagaccagagctaaggaagtgacatcacatggaacaatttgtgaacagcaagcagtagggcctggctgcaggacagggtgtgaagtgggggagcagtgatcaggagggccagagagatcagcagggatgtgatcttgagaagctgtgtgtgccatgatctggccctattaatccagaagggtctgatggaagcctctgtgattctcttccatggttaaacattttaattgtattatacctcggatattcctaaatatttaaaacactggcatggttgaactagacaacctttaagtagtttgttccaaccatgagatttagatttcatgatttaggttttatgatcttaaactgaaacctgttagttttctaccactagtgagatcatggcctctgcttttctcctgggaagtccctcttataatcactctcttcccatgattaaagggctactctgccttcatgttgctacccgctcccctggaaatggagaatcaagcaaggatgcggttttccttccattactacatccatacaagagtaaatcaagaataaaagtccagttaatgaaaagatcactggtcttaatatacttagcaaaattttaaaggcaattaaaagtatatacatagacaatgatcaaaattctaatgaaaagacccggctctcccctaaaagaagaaaaaatcatgtaatgtatatatgcattccataaaaacatacatggggaaaacttcagaagcctaaaaacaaaacatcagtaaaccaagccacacttagaaaaatgaaagctgatttttattttatcatcaacagccattctttagacatgaacatgcatacgtaatattctacgcacacatcacagcttttaacgttagttaataaaggttaaacacacaacatacatccttacaaaaaaagtcaaaatgcaaacttaaaactttaaacaaaagtattactaatttaaaaaaagtttgtgttgggtaccatttgtacaacacagttaatttaaacattttcattttggttgcacatgaaaaaggcggcagtagaaaataaagtcattgagggtttttaaatagcagaataggcagttttgccatgcaggagaagcaatattaaatattagtttcaaaaaaaatccacatttaaaaatatttagttcaagtcacagaatttttctcagtagagaccccaatgcaatgcataattagctgccttagatggcccgtttgaaaggatgatatcccttcagagtgtaactttactgattttggcacagaaaagaagtcttaagaacatgattaaaaaagagggaagaggaacagaggaaagaaataaaagcaagaataaatgagatagtaattgcaatcactaaaaaactgcattctcagtcattgcagaatactgtcttctgtctacagcaggtgcttattccagaattgttattgcagcatggatttaatttgcttggaggtagtctcatcattcaaatgttttgttgtgtacctgagagcatttagaagaccttccacactattaggaggttggtccttaagaactttgatacaacctttcatatcaattttggaagttttagcaaatgctcccactggatgtacgtggtcatagagtattatgacacccaccattaccctcaagcagaatgacactgtctcttcatttgtaaatctgcttctgtattccggtgtttccagcatgactctgcatacactagccattgtgcttaaacaatctgtggtattttctattggtaaatttttattctctgatacaaattttgttgtggcatcactcaaggttttcagcattggagttgcctcagcataaaacaaagacattcgatttgccaattcattatttacttcattttctccttctgccggtacattgttaatcctcatacgactcaatgttcttctataatagctgaaatcattctgtatggcaggatttgtcatcttgagttcatcaaaccggagtgtgaaatgaagaatttctgcaaactgtttagcaagagcctgctctcgctctagatgctgggtgggagaatatggggtacttgttaaggctcccagaagacctcttaatgctgcttctaacctctgagaaaattcgtaaaatttctttaatttgcctactagtggaacaactgcaccccatgccttctcttgcaacttctcatctgctggatgctggattgcctctcgtatttcgtggccagctcctctgtatgactgcaagtcctccaagatgccttctgcatcttttaatactacattcacctgattataaatttccttctcagactctgtaggctgggcattttcaaaatcaaggaaaaaatttggcccctgctcaaggtctgtgcatgtcaaaactttaagaagattccccatgttaaggtaccttcagccagtgctggtgattctgtccttgtccttctatcctccgctcgagcctccaggcgctctcagtcccgctcctgcgccctcctggagccgcagaggcggctcctcagcggcgctagggggagccccgggtccggagcgggggagcggcggcagccggaccgggagcccctcaacacctgcccctgtggcagagccgcgacaagccaggcggcagctccgagcggggagggcaagtgac

SEQ ID NO: 18485 - RNA, 3306 nt, Homo sapiens
  source 1..3306: mol_type = other RNA
tgagctgctgtaccaaaataccacaaactgcatggcttaaaacaacagaaatttattccctcacaatcctggaggccagatgtctgaaatcaagatattggtagggttggttccttctcgagactctgagggagaatctgtgacatgcctgttttcctagcttctagtgacttcctccaattcttagggttctttggctcatagatgcattgctctaatctctgcctccatcttcccatggccttcagctctgtgtgtctatttccccttcttttctaagagctagtcattgaatttagggcccaccctactacaggttgatctcatttccaggtccttgatttcatctgcaaaaactttttccaaataatgtcacacgtggagattcccagtgaatgtatctcctgggggccactattcagcctattacactattcttagaagatgcctagaaggatatggccaatgttatccagaaggcttcatgaaggaggtaatagaagctaacccttcaaagatgaaagttggcgttcattagagggtcacaaggggaggaagggaatgtcaggttcagggaccagccagaccagagctaaggaagtgacatcacatggaacaatttgtgaacagcaagcagtagggcctggctgcaggacagggtgtgaagtgggggagcagtgatcaggagggccagagagatcagcagggatgtgatcttgagaagctgtgtgtgccatgatctggccctattaatccagaagggtctgatggaagcctctgtgattctcttccatggttaaacattttaattgtattatacctcggatattcctaaatatttaaaacactggcatggttgaactagacaacctttaagtagtttgttccaaccatgagatttagatttcatgatttaggttttatgatcttaaactgaaacctgttagttttctaccactagtgagatcatggcctctgcttttctcctgggaagtccctcttataatcactctcttcccatgattaaagggctactctgccttcatgttgctacccgctcccctggaaatggagaatcaagcaaggatgcggttttccttccattactacatccatacaagagtaaatcaagaataaaagtccagttaatgaaaagatcactggtcttaatatacttagcaaaattttaaaggcaattaaaagtatatacatagacaatgatcaaaattctaatgaaaagacccggctctcccctaaaagaagaaaaaatcatgtaatgtatatatgcattccataaaaacatacatggggaaaacttcagaagcctaaaaacaaaacatcagtaaaccaagccacacttagaaaaatgaaagctgatttttattttatcatcaacagccattctttagacatgaacatgcatacgtaatattctacgcacacatcacagcttttaacgttagttaataaaggttaaacacacaacatacatccttacaaaaaaagtcaaaatgcaaacttaaaactttaaacaaaagtattactaatttaaaaaaagtttgtgttgggtaccatttgtacaacacagttaatttaaacattttcattttggttgcacatgaaaaaggcggcagtagaaaataaagtcattgagggtttttaaatagcagaataggcagttttgccatgcaggagaagcaatattaaatattagtttcaaaaaaaatccacatttaaaaatatttagttcaagtcacagaatttttctcagtagagaccccaatgcaatgcataattagctgccttagatggcccgtttgaaaggatgatatcccttcagagtgtaactttactgattttggcacagaaaagaagtcttaagaacatgattaaaaaagagggaagaggaacagaggaaagaaataaaagcaagaataaatgagatagtaattgcaatcactaaaaaactgcattctcagtcattgcagaatactgtcttctgtctacagcaggtgcttattccagaattgttattgcagcatggatttaatttgcttggaggtagtctcatcattcaaatgttttgttgtgtacctgagagcatttagaagaccttccacactattaggaggttggtccttaagaactttgatacaacctttcatatcaattttggaagttttagcaaatgctcccactggatgtacgtggtcatagagtattatgacacccaccattaccctcaagcagaatgacactgtctcttcatttgtaaatctgcttctgtattccggtgtttccagcatgactctgcatacactagccattgtgcttaaacaatctgtggtattttctattggtaaatttttattctctgatacaaattttgttgtggcatcactcaaggttttcagcattggagttgcctcagcataaaacaaagacattcgatttgccaattcattatttacttcattttctccttctgccggtacattgttaatcctcatacgactcaatgttcttctataatagctgaaatcattctgtatggcaggatttgtcatcttgagttcatcaaaccggagtgtgaaatgaagaatttctgcaaactgtttagcaagagcctgctctcgctctagatgctgggtgggagaatatggggtacttgttaaggctcccagaagacctcttaatgctgcttctaacctctgagaaaattcgtaaaatttctttaatttgcctactagtggaacaactgcaccccatgccttctcttgcaacttctcatctgctggatgctggattgcctctcgtatttcgtggccagctcctctgtatgactgcaagtcctccaagatgccttctgcatcttttaatactacattcacctgattataaatttccttctcagactctgtaggctgggcattttcaaaatcaaggaaaaaatttggcccctgctcaaggtctgtgcatgtcaaaactttaagaagattccccatgttaaggtaccttcagccagtgctggtgattctgtccttgtccttctatccttggattggcgttccctctttcctagttcacttgttccagtccttcaacttctgtttcttgctaacaggtgtgcaaatgaattaccaactgggtaaccttgaatgagttaatcaaattccaggcctcagtttcttctcctggacttcaggaatggtgacagcccctgcctggctcacctcgcagcggggtcagtgagaggaatgctgtccacgcacccattcagccctcccgcagatacttactgggcct

SEQ ID NO: 18486 - RNA, 3385 nt, Homo sapiens
  source 1..3385: mol_type = other RNA
tgagctgctgtaccaaaataccacaaactgcatggcttaaaacaacagaaatttattccctcacaatcctggaggccagatgtctgaaatcaagatattggtagggttggttccttctcgagactctgagggagaatctgtgacatgcctgttttcctagcttctagtgacttcctccaattcttagggttctttggctcatagatgcattgctctaatctctgcctccatcttcccatggccttcagctctgtgtgtctatttccccttcttttctaagagctagtcattgaatttagggcccaccctactacaggttgatctcatttccaggtccttgatttcatctgcaaaaactttttccaaataatgtcacacgtggagattcccagtgaatgtatctcctgggggccactattcagcctattacactattcttagaagatgcctagaaggatatggccaatgttatccagaaggcttcatgaaggaggtaatagaagctaacccttcaaagatgaaagttggcgttcattagagggtcacaaggggaggaagggaatgtcaggttcagggaccagccagaccagagctaaggaagtgacatcacatggaacaatttgtgaacagcaagcagtagggcctggctgcaggacagggtgtgaagtgggggagcagtgatcaggagggccagagagatcagcagggatgtgatcttgagaagctgtgtgtgccatgatctggccctattaatccagaagggtctgatggaagcctctgtgattctcttccatggttaaacattttaattgtattatacctcggatattcctaaatatttaaaacactggcatggttgaactagacaacctttaagtagtttgttccaaccatgagatttagatttcatgatttaggttttatgatcttaaactgaaacctgttagttttctaccactagtgagatcatggcctctgcttttctcctgggaagtccctcttataatcactctcttcccatgattaaagggctactctgccttcatgttgctacccgctcccctggaaatggagaatcaagcaaggatgcggttttccttccattactacatccatacaagagtaaatcaagaataaaagtccagttaatgaaaagatcactggtcttaatatacttagcaaaattttaaaggcaattaaaagtatatacatagacaatgatcaaaattctaatgaaaagacccggctctcccctaaaagaagaaaaaatcatgtaatgtatatatgcattccataaaaacatacatggggaaaacttcagaagcctaaaaacaaaacatcagtaaaccaagccacacttagaaaaatgaaagctgatttttattttatcatcaacagccattctttagacatgaacatgcatacgtaatattctacgcacacatcacagcttttaacgttagttaataaaggttaaacacacaacatacatccttacaaaaaaagtcaaaatgcaaacttaaaactttaaacaaaagtattactaatttaaaaaaagtttgtgttgggtaccatttgtacaacacagttaatttaaacattttcattttggttgcacatgaaaaaggcggcagtagaaaataaagtcattgagggtttttaaatagcagaataggcagttttgccatgcaggagaagcaatattaaatattagtttcaaaaaaaatccacatttaaaaatatttagttcaagtcacagaatttttctcagtagagaccccaatgcaatgcataattagctgccttagatggcccgtttgaaaggatgatatcccttcagagtgtaactttactgattttggcacagaaaagaagtcttaagaacatgattaaaaaagagggaagaggaacagaggaaagaaataaaagcaagaataaatgagatagtaattgcaatcactaaaaaactgcattctcagtcattgcagaatactgtcttctgtctacagcaggtgcttattccagaattgttattgcagcatggatttaatttgcttggaggtagtctcatcattcaaatgttttgttgtgtacctgagagcatttagaagaccttccacactattaggaggttggtccttaagaactttgatacaacctttcatatcaattttggaagttttagcaaatgctcccactggatgtacgtggtcatagagtattatgacacccaccattaccctcaagcagaatgacactgtctcttcatttgtaaatctgcttctgtattccggtgtttccagcatgactctgcatacactagccattgtgcttaaacaatctgtggtattttctattggtaaatttttattctctgatacaaattttgttgtggcatcactcaaggttttcagcattggagttgcctcagcataaaacaaagacattcgatttgccaattcattatttacttcattttctccttctgccggtacattgttaatcctcatacgactcaatgttcttctataatagctgaaatcattctgtatggcaggatttgtcatcttgagttcatcaaaccggagtgtgaaatgaagaatttctgcaaactgtttagcaagagcctgctctcgctctagatgctgggtgggagaatatggggtacttgttaaggctcccagaagacctcttaatgctgcttctaacctctgagaaaattcgtaaaatttctttaatttgcctactagtggaacaactgcaccccatgccttctcttgcaacttctcatctgctggatgctggattgcctctcgtatttcgtggccagctcctctgtatgactgcaagtcctccaagatgccttctgcatcttttaatactacattcacctgattataaatttccttctcagactctgtaggctgggcattttcaaaatcaaggaaaaaatttggcccctgctcaaggtctgtgcatgtcaaaactttaagaagattccccatgttaaggtaccttcagccagtgctggtgattctgtccttgtccttctatccttggattggcgttccctctttcctagttcacttgttccagtccttcaacttctgtttcttgctaacaggtgtgcaaatgaattaccaactgggtaaccttgaatgagttaatcaaattccaggcctcagtttcttctcctggcggcccgggcgggcgaggggagcgcggcgcgggagcgcaggagcctcggagcctccggtgccgccgccgccgccgtttccgggttggcggggctcacgtcaccgccacaggtttgcgagctgcccccgccgcggcggcagcagcagcagcagcagcagcccgggcgagtgccaggcgagaaataact

SEQ ID NO: 18487 - RNA, 3285 nt, Homo sapiens
  source 1..3285: mol_type = other RNA
tgagctgctgtaccaaaataccacaaactgcatggcttaaaacaacagaaatttattccctcacaatcctggaggccagatgtctgaaatcaagatattggtagggttggttccttctcgagactctgagggagaatctgtgacatgcctgttttcctagcttctagtgacttcctccaattcttagggttctttggctcatagatgcattgctctaatctctgcctccatcttcccatggccttcagctctgtgtgtctatttccccttcttttctaagagctagtcattgaatttagggcccaccctactacaggttgatctcatttccaggtccttgatttcatctgcaaaaactttttccaaataatgtcacacgtggagattcccagtgaatgtatctcctgggggccactattcagcctattacactattcttagaagatgcctagaaggatatggccaatgttatccagaaggcttcatgaaggaggtaatagaagctaacccttcaaagatgaaagttggcgttcattagagggtcacaaggggaggaagggaatgtcaggttcagggaccagccagaccagagctaaggaagtgacatcacatggaacaatttgtgaacagcaagcagtagggcctggctgcaggacagggtgtgaagtgggggagcagtgatcaggagggccagagagatcagcagggatgtgatcttgagaagctgtgtgtgccatgatctggccctattaatccagaagggtctgatggaagcctctgtgattctcttccatggttaaacattttaattgtattatacctcggatattcctaaatatttaaaacactggcatggttgaactagacaacctttaagtagtttgttccaaccatgagatttagatttcatgatttaggttttatgatcttaaactgaaacctgttagttttctaccactagtgagatcatggcctctgcttttctcctgggaagtccctcttataatcactctcttcccatgattaaagggctactctgccttcatgttgctacccgctcccctggaaatggagaatcaagcaaggatgcggttttccttccattactacatccatacaagagtaaatcaagaataaaagtccagttaatgaaaagatcactggtcttaatatacttagcaaaattttaaaggcaattaaaagtatatacatagacaatgatcaaaattctaatgaaaagacccggctctcccctaaaagaagaaaaaatcatgtaatgtatatatgcattccataaaaacatacatggggaaaacttcagaagcctaaaaacaaaacatcagtaaaccaagccacacttagaaaaatgaaagctgatttttattttatcatcaacagccattctttagacatgaacatgcatacgtaatattctacgcacacatcacagcttttaacgttagttaataaaggttaaacacacaacatacatccttacaaaaaaagtcaaaatgcaaacttaaaactttaaacaaaagtattactaatttaaaaaaagtttgtgttgggtaccatttgtacaacacagttaatttaaacattttcattttggttgcacatgaaaaaggcggcagtagaaaataaagtcattgagggtttttaaatagcagaataggcagttttgccatgcaggagaagcaatattaaatattagtttcaaaaaaaatccacatttaaaaatatttagttcaagtcacagaatttttctcagtagagaccccaatgcaatgcataattagctgccttagatggcccgtttgaaaggatgatatcccttcagagtgtaactttactgattttggcacagaaaagaagtcttaagaacatgattaaaaaagagggaagaggaacagaggaaagaaataaaagcaagaataaatgagatagtaattgcaatcactaaaaaactgcattctcagtcattgcagaatactgtcttctgtctacagcaggtgcttattccagaattgttattgcagcatggatttaatttgcttggaggtagtctcatcattcaaatgttttgttgtgtacctgagagcatttagaagaccttccacactattaggaggttggtccttaagaactttgatacaacctttcatatcaattttggaagttttagcaaatgctcccactggatgtacgtggtcatagagtattatgacacccaccattaccctcaagcagaatgacactgtctcttcatttgtaaatctgcttctgtattccggtgtttccagcatgactctgcatacactagccattgtgcttaaacaatctgtggtattttctattggtaaatttttattctctgatacaaattttgttgtggcatcactcaaggttttcagcattggagttgcctcagcataaaacaaagacattcgatttgccaattcattatttacttcattttctccttctgccggtacattgttaatcctcatacgactcaatgttcttctataatagctgaaatcattctgtatggcaggatttgtcatcttgagttcatcaaaccggagtgtgaaatgaagaatttctgcaaactgtttagcaagagcctgctctcgctctagatgctgggtgggagaatatggggtacttgttaaggctcccagaagacctcttaatgctgcttctaacctctgagaaaattcgtaaaatttctttaatttgcctactagtggaacaactgcaccccatgccttctcttgcaacttctcatctgctggatgctggattgcctctcgtatttcgtggccagctcctctgtatgactgcaagtcctccaagatgccttctgcatcttttaatactacattcacctgattataaatttccttctcagactctgtaggctgggcattttcaaaatcaaggaaaaaatttggcccctgctcaaggtctgtgcatgtcaaaactttaagaagattccccatgttaaggtaccttcagccagtgctggtgattctgtccttgtccttctatccttggattggcgttccctctttcctagttcacttgttccagtccttcaacttctgtttcttgctaacaggtgtgcaaatgaattaccaactgggtaaccttgaatgagttaatcaaattccaggcctcagtttcttctccttcgagaagccgagccgccggcgctcgcacaaaaggaggacgctcgcctcgcgacgcgcctccccccgcgcccagtccccgccgcatcgc

SEQ ID NO: 18488 - RNA, 3345 nt, Homo sapiens
  source 1..3345: mol_type = other RNA
tgagctgctgtaccaaaataccacaaactgcatggcttaaaacaacagaaatttattccctcacaatcctggaggccagatgtctgaaatcaagatattggtagggttggttccttctcgagactctgagggagaatctgtgacatgcctgttttcctagcttctagtgacttcctccaattcttagggttctttggctcatagatgcattgctctaatctctgcctccatcttcccatggccttcagctctgtgtgtctatttccccttcttttctaagagctagtcattgaatttagggcccaccctactacaggttgatctcatttccaggtccttgatttcatctgcaaaaactttttccaaataatgtcacacgtggagattcccagtgaatgtatctcctgggggccactattcagcctattacactattcttagaagatgcctagaaggatatggccaatgttatccagaaggcttcatgaaggaggtaatagaagctaacccttcaaagatgaaagttggcgttcattagagggtcacaaggggaggaagggaatgtcaggttcagggaccagccagaccagagctaaggaagtgacatcacatggaacaatttgtgaacagcaagcagtagggcctggctgcaggacagggtgtgaagtgggggagcagtgatcaggagggccagagagatcagcagggatgtgatcttgagaagctgtgtgtgccatgatctggccctattaatccagaagggtctgatggaagcctctgtgattctcttccatggttaaacattttaattgtattatacctcggatattcctaaatatttaaaacactggcatggttgaactagacaacctttaagtagtttgttccaaccatgagatttagatttcatgatttaggttttatgatcttaaactgaaacctgttagttttctaccactagtgagatcatggcctctgcttttctcctgggaagtccctcttataatcactctcttcccatgattaaagggctactctgccttcatgttgctacccgctcccctggaaatggagaatcaagcaaggatgcggttttccttccattactacatccatacaagagtaaatcaagaataaaagtccagttaatgaaaagatcactggtcttaatatacttagcaaaattttaaaggcaattaaaagtatatacatagacaatgatcaaaattctaatgaaaagacccggctctcccctaaaagaagaaaaaatcatgtaatgtatatatgcattccataaaaacatacatggggaaaacttcagaagcctaaaaacaaaacatcagtaaaccaagccacacttagaaaaatgaaagctgatttttattttatcatcaacagccattctttagacatgaacatgcatacgtaatattctacgcacacatcacagcttttaacgttagttaataaaggttaaacacacaacatacatccttacaaaaaaagtcaaaatgcaaacttaaaactttaaacaaaagtattactaatttaaaaaaagtttgtgttgggtaccatttgtacaacacagttaatttaaacattttcattttggttgcacatgaaaaaggcggcagtagaaaataaagtcattgagggtttttaaatagcagaataggcagttttgccatgcaggagaagcaatattaaatattagtttcaaaaaaaatccacatttaaaaatatttagttcaagtcacagaatttttctcagtagagaccccaatgcaatgcataattagctgccttagatggcccgtttgaaaggatgatatcccttcagagtgtaactttactgattttggcacagaaaagaagtcttaagaacatgattaaaaaagagggaagaggaacagaggaaagaaataaaagcaagaataaatgagatagtaattgcaatcactaaaaaactgcattctcagtcattgcagaatactgtcttctgtctacagcaggtgcttattccagaattgttattgcagcatggatttaatttgcttggaggtagtctcatcattcaaatgttttgttgtgtacctgagagcatttagaagaccttccacactattaggaggttggtccttaagaactttgatacaacctttcatatcaattttggaagttttagcaaatgctcccactggatgtacgtggtcatagagtattatgacacccaccattaccctcaagcagaatgacactgtctcttcatttgtaaatctgcttctgtattccggtgtttccagcatgactctgcatacactagccattgtgcttaaacaatctgtggtattttctattggtaaatttttattctctgatacaaattttgttgtggcatcactcaaggttttcagcattggagttgcctcagcataaaacaaagacattcgatttgccaattcattatttacttcattttctccttctgccggtacattgttaatcctcatacgactcaatgttcttctataatagctgaaatcattctgtatggcaggatttgtcatcttgagttcatcaaaccggagtgtgaaatgaagaatttctgcaaactgtttagcaagagcctgctctcgctctagatgctgggtgggagaatatggggtacttgttaaggctcccagaagacctcttaatgctgcttctaacctctgagaaaattcgtaaaatttctttaatttgcctactagtggaacaactgcaccccatgccttctcttgcaacttctcatctgctggatgctggattgcctctcgtatttcgtggccagctcctctgtatgactgcaagtcctccaagatgccttctgcatcttttaatactacattcacctgattataaatttccttctcagactctgtaggctgggcattttcaaaatcaaggaaaaaatttggcccctgctcaaggtctgtgcatgtcaaaactttaagaagattccccatgttaaggtaccttcagccagtgctggtgattctgtccttgtccttctatccttggattggcgttccctctttcctagttcacttgttccagtccttcaacttctgtttcttgctaacaggtgtgcaaatgaattaccctccgctcgagcctccaggcgctctcagtcccgctcctgcgccctcctggagccgcagaggcggctcctcagcggcgctagggggagccccgggtccggagcgggggagcggcggcagccggaccgggagcccctcaacacctgcccctgtggcagagccgcgacaagccaggcggcagctccgagcggggagggcaagtgac

SEQ ID NO: 18489 - RNA, 3431 nt, Homo sapiens
  source 1..3431: mol_type = other RNA
tgagctgctgtaccaaaataccacaaactgcatggcttaaaacaacagaaatttattccctcacaatcctggaggccagatgtctgaaatcaagatattggtagggttggttccttctcgagactctgagggagaatctgtgacatgcctgttttcctagcttctagtgacttcctccaattcttagggttctttggctcatagatgcattgctctaatctctgcctccatcttcccatggccttcagctctgtgtgtctatttccccttcttttctaagagctagtcattgaatttagggcccaccctactacaggttgatctcatttccaggtccttgatttcatctgcaaaaactttttccaaataatgtcacacgtggagattcccagtgaatgtatctcctgggggccactattcagcctattacactattcttagaagatgcctagaaggatatggccaatgttatccagaaggcttcatgaaggaggtaatagaagctaacccttcaaagatgaaagttggcgttcattagagggtcacaaggggaggaagggaatgtcaggttcagggaccagccagaccagagctaaggaagtgacatcacatggaacaatttgtgaacagcaagcagtagggcctggctgcaggacagggtgtgaagtgggggagcagtgatcaggagggccagagagatcagcagggatgtgatcttgagaagctgtgtgtgccatgatctggccctattaatccagaagggtctgatggaagcctctgtgattctcttccatggttaaacattttaattgtattatacctcggatattcctaaatatttaaaacactggcatggttgaactagacaacctttaagtagtttgttccaaccatgagatttagatttcatgatttaggttttatgatcttaaactgaaacctgttagttttctaccactagtgagatcatggcctctgcttttctcctgggaagtccctcttataatcactctcttcccatgattaaagggctactctgccttcatgttgctacccgctcccctggaaatggagaatcaagcaaggatgcggttttccttccattactacatccatacaagagtaaatcaagaataaaagtccagttaatgaaaagatcactggtcttaatatacttagcaaaattttaaaggcaattaaaagtatatacatagacaatgatcaaaattctaatgaaaagacccggctctcccctaaaagaagaaaaaatcatgtaatgtatatatgcattccataaaaacatacatggggaaaacttcagaagcctaaaaacaaaacatcagtaaaccaagccacacttagaaaaatgaaagctgatttttattttatcatcaacagccattctttagacatgaacatgcatacgtaatattctacgcacacatcacagcttttaacgttagttaataaaggttaaacacacaacatacatccttacaaaaaaagtcaaaatgcaaacttaaaactttaaacaaaagtattactaatttaaaaaaagtttgtgttgggtaccatttgtacaacacagttaatttaaacattttcattttggttgcacatgaaaaaggcggcagtagaaaataaagtcattgagggtttttaaatagcagaataggcagttttgccatgcaggagaagcaatattaaatattagtttcaaaaaaaatccacatttaaaaatatttagttcaagtcacagaatttttctcagtagagaccccaatgcaatgcataattagctgccttagatggcccgtttgaaaggatgatatcccttcagagtgtaactttactgattttggcacagaaaagaagtcttaagaacatgattaaaaaagagggaagaggaacagaggaaagaaataaaagcaagaataaatgagatagtaattgcaatcactaaaaaactgcattctcagtcattgcagaatactgtcttctgtctacagcaggtgcttattccagaattgttattgcagcatggatttaatttgcttggaggtagtctcatcattcaaatgttttgttgtgtacctgagagcatttagaagaccttccacactattaggaggttggtccttaagaactttgatacaacctttcatatcaattttggaagttttagcaaatgctcccactggatgtacgtggtcatagagtattatgacacccaccattaccctcaagcagaatgacactgtctcttcatttgtaaatctgcttctgtattccggtgtttccagcatgactctgcatacactagccattgtgcttaaacaatctgtggtattttctattggtaaatttttattctctgatacaaattttgttgtggcatcactcaaggttttcagcattggagttgcctcagcataaaacaaagacattcgatttgccaattcattatttacttcattttctccttctgccggtacattgttaatcctcatacgactcaatgttcttctataatagctgaaatcattctgtatggcaggatttgtcatcttgagttcatcaaaccggagtgtgaaatgaagaatttctgcaaactgtttagcaagagcctgctctcgctctagatgctgggtgggagaatatggggtacttgttaaggctcccagaagacctcttaatgctgcttctaacctctgagaaaattcgtaaaatttctttaatttgcctactagtggaacaactgcaccccatgccttctcttgcaacttctcatctgctggatgctggattgcctctcgtatttcgtggccagctcctctgtatgactgcaagtcctccaagatgccttctgcatcttttaatactacattcacctgattataaatttccttctcagactctgtaggctgggcattttcaaaatcaaggaaaaaatttggcccctgctcaaggtctgtgcatgtcaaaactttaagaagattccccatgttaaggtaccttcagccagtgctggtgattctgtccttgtccttctatccttggattggcgttccctctttcctagttcacttgttccagtccttcaacttctgtttcttgctaacaggtgtgcaaatgaattacctgagaagtgcaaggttggttcagaatacctactgttttcaccacccaactgggtaaccttgaatgagttaatcaaattccaggcctcagtttcttctcctggcggcccgggcgggcgaggggagcgcggcgcgggagcgcaggagcctcggagcctccggtgccgccgccgccgccgtttccgggttggcggggctcacgtcaccgccacaggtttgcgagctgcccccgccgcggcggcagcagcagcagcagcagcagcccgggcgagtgccaggcgagaaataact

SEQ ID NO: 18490 - RNA, 3331 nt, Homo sapiens
  source 1..3331: mol_type = other RNA
tgagctgctgtaccaaaataccacaaactgcatggcttaaaacaacagaaatttattccctcacaatcctggaggccagatgtctgaaatcaagatattggtagggttggttccttctcgagactctgagggagaatctgtgacatgcctgttttcctagcttctagtgacttcctccaattcttagggttctttggctcatagatgcattgctctaatctctgcctccatcttcccatggccttcagctctgtgtgtctatttccccttcttttctaagagctagtcattgaatttagggcccaccctactacaggttgatctcatttccaggtccttgatttcatctgcaaaaactttttccaaataatgtcacacgtggagattcccagtgaatgtatctcctgggggccactattcagcctattacactattcttagaagatgcctagaaggatatggccaatgttatccagaaggcttcatgaaggaggtaatagaagctaacccttcaaagatgaaagttggcgttcattagagggtcacaaggggaggaagggaatgtcaggttcagggaccagccagaccagagctaaggaagtgacatcacatggaacaatttgtgaacagcaagcagtagggcctggctgcaggacagggtgtgaagtgggggagcagtgatcaggagggccagagagatcagcagggatgtgatcttgagaagctgtgtgtgccatgatctggccctattaatccagaagggtctgatggaagcctctgtgattctcttccatggttaaacattttaattgtattatacctcggatattcctaaatatttaaaacactggcatggttgaactagacaacctttaagtagtttgttccaaccatgagatttagatttcatgatttaggttttatgatcttaaactgaaacctgttagttttctaccactagtgagatcatggcctctgcttttctcctgggaagtccctcttataatcactctcttcccatgattaaagggctactctgccttcatgttgctacccgctcccctggaaatggagaatcaagcaaggatgcggttttccttccattactacatccatacaagagtaaatcaagaataaaagtccagttaatgaaaagatcactggtcttaatatacttagcaaaattttaaaggcaattaaaagtatatacatagacaatgatcaaaattctaatgaaaagacccggctctcccctaaaagaagaaaaaatcatgtaatgtatatatgcattccataaaaacatacatggggaaaacttcagaagcctaaaaacaaaacatcagtaaaccaagccacacttagaaaaatgaaagctgatttttattttatcatcaacagccattctttagacatgaacatgcatacgtaatattctacgcacacatcacagcttttaacgttagttaataaaggttaaacacacaacatacatccttacaaaaaaagtcaaaatgcaaacttaaaactttaaacaaaagtattactaatttaaaaaaagtttgtgttgggtaccatttgtacaacacagttaatttaaacattttcattttggttgcacatgaaaaaggcggcagtagaaaataaagtcattgagggtttttaaatagcagaataggcagttttgccatgcaggagaagcaatattaaatattagtttcaaaaaaaatccacatttaaaaatatttagttcaagtcacagaatttttctcagtagagaccccaatgcaatgcataattagctgccttagatggcccgtttgaaaggatgatatcccttcagagtgtaactttactgattttggcacagaaaagaagtcttaagaacatgattaaaaaagagggaagaggaacagaggaaagaaataaaagcaagaataaatgagatagtaattgcaatcactaaaaaactgcattctcagtcattgcagaatactgtcttctgtctacagcaggtgcttattccagaattgttattgcagcatggatttaatttgcttggaggtagtctcatcattcaaatgttttgttgtgtacctgagagcatttagaagaccttccacactattaggaggttggtccttaagaactttgatacaacctttcatatcaattttggaagttttagcaaatgctcccactggatgtacgtggtcatagagtattatgacacccaccattaccctcaagcagaatgacactgtctcttcatttgtaaatctgcttctgtattccggtgtttccagcatgactctgcatacactagccattgtgcttaaacaatctgtggtattttctattggtaaatttttattctctgatacaaattttgttgtggcatcactcaaggttttcagcattggagttgcctcagcataaaacaaagacattcgatttgccaattcattatttacttcattttctccttctgccggtacattgttaatcctcatacgactcaatgttcttctataatagctgaaatcattctgtatggcaggatttgtcatcttgagttcatcaaaccggagtgtgaaatgaagaatttctgcaaactgtttagcaagagcctgctctcgctctagatgctgggtgggagaatatggggtacttgttaaggctcccagaagacctcttaatgctgcttctaacctctgagaaaattcgtaaaatttctttaatttgcctactagtggaacaactgcaccccatgccttctcttgcaacttctcatctgctggatgctggattgcctctcgtatttcgtggccagctcctctgtatgactgcaagtcctccaagatgccttctgcatcttttaatactacattcacctgattataaatttccttctcagactctgtaggctgggcattttcaaaatcaaggaaaaaatttggcccctgctcaaggtctgtgcatgtcaaaactttaagaagattccccatgttaaggtaccttcagccagtgctggtgattctgtccttgtccttctatccttggattggcgttccctctttcctagttcacttgttccagtccttcaacttctgtttcttgctaacaggtgtgcaaatgaattacctgagaagtgcaaggttggttcagaatacctactgttttcaccacccaactgggtaaccttgaatgagttaatcaaattccaggcctcagtttcttctccttcgagaagccgagccgccggcgctcgcacaaaaggaggacgctcgcctcgcgacgcgcctccccccgcgcccagtccccgccgcatcgc

SEQ ID NO: 18491 - RNA, 3332 nt, Homo sapiens
  source 1..3332: mol_type = other RNA
tgagctgctgtaccaaaataccacaaactgcatggcttaaaacaacagaaatttattccctcacaatcctggaggccagatgtctgaaatcaagatattggtagggttggttccttctcgagactctgagggagaatctgtgacatgcctgttttcctagcttctagtgacttcctccaattcttagggttctttggctcatagatgcattgctctaatctctgcctccatcttcccatggccttcagctctgtgtgtctatttccccttcttttctaagagctagtcattgaatttagggcccaccctactacaggttgatctcatttccaggtccttgatttcatctgcaaaaactttttccaaataatgtcacacgtggagattcccagtgaatgtatctcctgggggccactattcagcctattacactattcttagaagatgcctagaaggatatggccaatgttatccagaaggcttcatgaaggaggtaatagaagctaacccttcaaagatgaaagttggcgttcattagagggtcacaaggggaggaagggaatgtcaggttcagggaccagccagaccagagctaaggaagtgacatcacatggaacaatttgtgaacagcaagcagtagggcctggctgcaggacagggtgtgaagtgggggagcagtgatcaggagggccagagagatcagcagggatgtgatcttgagaagctgtgtgtgccatgatctggccctattaatccagaagggtctgatggaagcctctgtgattctcttccatggttaaacattttaattgtattatacctcggatattcctaaatatttaaaacactggcatggttgaactagacaacctttaagtagtttgttccaaccatgagatttagatttcatgatttaggttttatgatcttaaactgaaacctgttagttttctaccactagtgagatcatggcctctgcttttctcctgggaagtccctcttataatcactctcttcccatgattaaagggctactctgccttcatgttgctacccgctcccctggaaatggagaatcaagcaaggatgcggttttccttccattactacatccatacaagagtaaatcaagaataaaagtccagttaatgaaaagatcactggtcttaatatacttagcaaaattttaaaggcaattaaaagtatatacatagacaatgatcaaaattctaatgaaaagacccggctctcccctaaaagaagaaaaaatcatgtaatgtatatatgcattccataaaaacatacatggggaaaacttcagaagcctaaaaacaaaacatcagtaaaccaagccacacttagaaaaatgaaagctgatttttattttatcatcaacagccattctttagacatgaacatgcatacgtaatattctacgcacacatcacagcttttaacgttagttaataaaggttaaacacacaacatacatccttacaaaaaaagtcaaaatgcaaacttaaaactttaaacaaaagtattactaatttaaaaaaagtttgtgttgggtaccatttgtacaacacagttaatttaaacattttcattttggttgcacatgaaaaaggcggcagtagaaaataaagtcattgagggtttttaaatagcagaataggcagttttgccatgcaggagaagcaatattaaatattagtttcaaaaaaaatccacatttaaaaatatttagttcaagtcacagaatttttctcagtagagaccccaatgcaatgcataattagctgccttagatggcccgtttgaaaggatgatatcccttcagagtgtaactttactgattttggcacagaaaagaagtcttaagaacatgattaaaaaagagggaagaggaacagaggaaagaaataaaagcaagaataaatgagatagtaattgcaatcactaaaaaactgcattctcagtcattgcagaatactgtcttctgtctacagcaggtgcttattccagaattgttattgcagcatggatttaatttgcttggaggtagtctcatcattcaaatgttttgttgtgtacctgagagcatttagaagaccttccacactattaggaggttggtccttaagaactttgatacaacctttcatatcaattttggaagttttagcaaatgctcccactggatgtacgtggtcatagagtattatgacacccaccattaccctcaagcagaatgacactgtctcttcatttgtaaatctgcttctgtattccggtgtttccagcatgactctgcatacactagccattgtgcttaaacaatctgtggtattttctattggtaaatttttattctctgatacaaattttgttgtggcatcactcaaggttttcagcattggagttgcctcagcataaaacaaagacattcgatttgccaattcattatttacttcattttctccttctgccggtacattgttaatcctcatacgactcaatgttcttctataatagctgaaatcattctgtatggcaggatttgtcatcttgagttcatcaaaccggagtgtgaaatgaagaatttctgcaaactgtttagcaagagcctgctctcgctctagatgctgggtgggagaatatggggtacttgttaaggctcccagaagacctcttaatgctgcttctaacctctgagaaaattcgtaaaatttctttaatttgcctactagtggaacaactgcaccccatgccttctcttgcaacttctcatctgctggatgctggattgcctctcgtatttcgtggccagctcctctgtatgactgcaagtcctccaagatgccttctgcatcttttaatactacattcacctgattataaatttccttctcagactctgtaggctgggcattttcaaaatcaaggaaaaaatttggcccctgctcaaggtctgtgcatgtcaaaactttaagaagattccccatgttaaggtaccttcagccagtgctggtgattctgtccttgtccttctatccttggattggcgttccctctttcctagttcacttgttccagtccttcaacttctgtttcttgctaacaggtgtgcaaatgaattacctggcggcccgggcgggcgaggggagcgcggcgcgggagcgcaggagcctcggagcctccggtgccgccgccgccgccgtttccgggttggcggggctcacgtcaccgccacaggtttgcgagctgcccccgccgcggcggcagcagcagcagcagcagcagcccgggcgagtgccaggcgagaaataact

SEQ ID NO: 18492 - RNA, 3232 nt, Homo sapiens
  source 1..3232: mol_type = other RNA
tgagctgctgtaccaaaataccacaaactgcatggcttaaaacaacagaaatttattccctcacaatcctggaggccagatgtctgaaatcaagatattggtagggttggttccttctcgagactctgagggagaatctgtgacatgcctgttttcctagcttctagtgacttcctccaattcttagggttctttggctcatagatgcattgctctaatctctgcctccatcttcccatggccttcagctctgtgtgtctatttccccttcttttctaagagctagtcattgaatttagggcccaccctactacaggttgatctcatttccaggtccttgatttcatctgcaaaaactttttccaaataatgtcacacgtggagattcccagtgaatgtatctcctgggggccactattcagcctattacactattcttagaagatgcctagaaggatatggccaatgttatccagaaggcttcatgaaggaggtaatagaagctaacccttcaaagatgaaagttggcgttcattagagggtcacaaggggaggaagggaatgtcaggttcagggaccagccagaccagagctaaggaagtgacatcacatggaacaatttgtgaacagcaagcagtagggcctggctgcaggacagggtgtgaagtgggggagcagtgatcaggagggccagagagatcagcagggatgtgatcttgagaagctgtgtgtgccatgatctggccctattaatccagaagggtctgatggaagcctctgtgattctcttccatggttaaacattttaattgtattatacctcggatattcctaaatatttaaaacactggcatggttgaactagacaacctttaagtagtttgttccaaccatgagatttagatttcatgatttaggttttatgatcttaaactgaaacctgttagttttctaccactagtgagatcatggcctctgcttttctcctgggaagtccctcttataatcactctcttcccatgattaaagggctactctgccttcatgttgctacccgctcccctggaaatggagaatcaagcaaggatgcggttttccttccattactacatccatacaagagtaaatcaagaataaaagtccagttaatgaaaagatcactggtcttaatatacttagcaaaattttaaaggcaattaaaagtatatacatagacaatgatcaaaattctaatgaaaagacccggctctcccctaaaagaagaaaaaatcatgtaatgtatatatgcattccataaaaacatacatggggaaaacttcagaagcctaaaaacaaaacatcagtaaaccaagccacacttagaaaaatgaaagctgatttttattttatcatcaacagccattctttagacatgaacatgcatacgtaatattctacgcacacatcacagcttttaacgttagttaataaaggttaaacacacaacatacatccttacaaaaaaagtcaaaatgcaaacttaaaactttaaacaaaagtattactaatttaaaaaaagtttgtgttgggtaccatttgtacaacacagttaatttaaacattttcattttggttgcacatgaaaaaggcggcagtagaaaataaagtcattgagggtttttaaatagcagaataggcagttttgccatgcaggagaagcaatattaaatattagtttcaaaaaaaatccacatttaaaaatatttagttcaagtcacagaatttttctcagtagagaccccaatgcaatgcataattagctgccttagatggcccgtttgaaaggatgatatcccttcagagtgtaactttactgattttggcacagaaaagaagtcttaagaacatgattaaaaaagagggaagaggaacagaggaaagaaataaaagcaagaataaatgagatagtaattgcaatcactaaaaaactgcattctcagtcattgcagaatactgtcttctgtctacagcaggtgcttattccagaattgttattgcagcatggatttaatttgcttggaggtagtctcatcattcaaatgttttgttgtgtacctgagagcatttagaagaccttccacactattaggaggttggtccttaagaactttgatacaacctttcatatcaattttggaagttttagcaaatgctcccactggatgtacgtggtcatagagtattatgacacccaccattaccctcaagcagaatgacactgtctcttcatttgtaaatctgcttctgtattccggtgtttccagcatgactctgcatacactagccattgtgcttaaacaatctgtggtattttctattggtaaatttttattctctgatacaaattttgttgtggcatcactcaaggttttcagcattggagttgcctcagcataaaacaaagacattcgatttgccaattcattatttacttcattttctccttctgccggtacattgttaatcctcatacgactcaatgttcttctataatagctgaaatcattctgtatggcaggatttgtcatcttgagttcatcaaaccggagtgtgaaatgaagaatttctgcaaactgtttagcaagagcctgctctcgctctagatgctgggtgggagaatatggggtacttgttaaggctcccagaagacctcttaatgctgcttctaacctctgagaaaattcgtaaaatttctttaatttgcctactagtggaacaactgcaccccatgccttctcttgcaacttctcatctgctggatgctggattgcctctcgtatttcgtggccagctcctctgtatgactgcaagtcctccaagatgccttctgcatcttttaatactacattcacctgattataaatttccttctcagactctgtaggctgggcattttcaaaatcaaggaaaaaatttggcccctgctcaaggtctgtgcatgtcaaaactttaagaagattccccatgttaaggtaccttcagccagtgctggtgattctgtccttgtccttctatccttggattggcgttccctctttcctagttcacttgttccagtccttcaacttctgtttcttgctaacaggtgtgcaaatgaattaccttcgagaagccgagccgccggcgctcgcacaaaaggaggacgctcgcctcgcgacgcgcctccccccgcgcccagtccccgccgcatcgc

SEQ ID NO: 18493 - RNA, 3344 nt, Homo sapiens
  source 1..3344: mol_type = other RNA
tgagctgctgtaccaaaataccacaaactgcatggcttaaaacaacagaaatttattccctcacaatcctggaggccagatgtctgaaatcaagatattggtagggttggttccttctcgagactctgagggagaatctgtgacatgcctgttttcctagcttctagtgacttcctccaattcttagggttctttggctcatagatgcattgctctaatctctgcctccatcttcccatggccttcagctctgtgtgtctatttccccttcttttctaagagctagtcattgaatttagggcccaccctactacaggttgatctcatttccaggtccttgatttcatctgcaaaaactttttccaaataatgtcacacgtggagattcccagtgaatgtatctcctgggggccactattcagcctattacactattcttagaagatgcctagaaggatatggccaatgttatccagaaggcttcatgaaggaggtaatagaagctaacccttcaaagatgaaagttggcgttcattagagggtcacaaggggaggaagggaatgtcaggttcagggaccagccagaccagagctaaggaagtgacatcacatggaacaatttgtgaacagcaagcagtagggcctggctgcaggacagggtgtgaagtgggggagcagtgatcaggagggccagagagatcagcagggatgtgatcttgagaagctgtgtgtgccatgatctggccctattaatccagaagggtctgatggaagcctctgtgattctcttccatggttaaacattttaattgtattatacctcggatattcctaaatatttaaaacactggcatggttgaactagacaacctttaagtagtttgttccaaccatgagatttagatttcatgatttaggttttatgatcttaaactgaaacctgttagttttctaccactagtgagatcatggcctctgcttttctcctgggaagtccctcttataatcactctcttcccatgattaaagggctactctgccttcatgttgctacccgctcccctggaaatggagaatcaagcaaggatgcggttttccttccattactacatccatacaagagtaaatcaagaataaaagtccagttaatgaaaagatcactggtcttaatatacttagcaaaattttaaaggcaattaaaagtatatacatagacaatgatcaaaattctaatgaaaagacccggctctcccctaaaagaagaaaaaatcatgtaatgtatatatgcattccataaaaacatacatggggaaaacttcagaagcctaaaaacaaaacatcagtaaaccaagccacacttagaaaaatgaaagctgatttttattttatcatcaacagccattctttagacatgaacatgcatacgtaatattctacgcacacatcacagcttttaacgttagttaataaaggttaaacacacaacatacatccttacaaaaaaagtcaaaatgcaaacttaaaactttaaacaaaagtattactaatttaaaaaaagtttgtgttgggtaccatttgtacaacacagttaatttaaacattttcattttggttgcacatgaaaaaggcggcagtagaaaataaagtcattgagggtttttaaatagcagaataggcagttttgccatgcaggagaagcaatattaaatattagtttcaaaaaaaatccacatttaaaaatatttagttcaagtcacagaatttttctcagtagagaccccaatgcaatgcataattagctgccttagatggcccgtttgaaaggatgatatcccttcagagtgtaactttactgattttggcacagaaaagaagtcttaagaacatgattaaaaaagagggaagaggaacagaggaaagaaataaaagcaagaataaatgagatagtaattgcaatcactaaaaaactgcattctcagtcattgcagaatactgtcttctgtctacagcaggtgcttattccagaattgttattgcagcatggatttaatttgcttggaggtagtctcatcattcaaatgttttgttgtgtacctgagagcatttagaagaccttccacactattaggaggttggtccttaagaactttgatacaacctttcatatcaattttggaagttttagcaaatgctcccactggatgtacgtggtcatagagtattatgacacccaccattaccctcaagcagaatgacactgtctcttcatttgtaaatctgcttctgtattccggtgtttccagcatgactctgcatacactagccattgtgcttaaacaatctgtggtattttctattggtaaatttttattctctgatacaaattttgttgtggcatcactcaaggttttcagcattggagttgcctcagcataaaacaaagacattcgatttgccaattcattatttacttcattttctccttctgccggtacattgttaatcctcatacgactcaatgttcttctataatagctgaaatcattctgtatggcaggatttgtcatcttgagttcatcaaaccggagtgtgaaatgaagaatttctgcaaactgtttagcaagagcctgctctcgctctagatgctgggtgggagaatatggggtacttgttaaggctcccagaagacctcttaatgctgcttctaacctctgagaaaattcgtaaaatttctttaatttgcctactagtggaacaactgcaccccatgccttctcttgcaacttctcatctgctggatgctggattgcctctcgtatttcgtggccagctcctctgtatgactgcaagtcctccaagatgccttctgcatcttttaatactacattcacctgattataaatttccttctcagactctgtaggctgggcattttcaaaatcaaggaaaaaatttggcccctgctcaaggtctgtgcatgtcaaaactttaagaagattccccatgttaaggtaccttcagccagtgctggtgattctgtccttgtccttctatctgagaagtgcaaggttggttcagaatacctactgttttcaccacccaactgggtaaccttgaatgagttaatcaaattccaggcctcagtttcttctcctggcggcccgggcgggcgaggggagcgcggcgcgggagcgcaggagcctcggagcctccggtgccgccgccgccgccgtttccgggttggcggggctcacgtcaccgccacaggtttgcgagctgcccccgccgcggcggcagcagcagcagcagcagcagcccgggcgagtgccaggcgagaaataact

SEQ ID NO: 18494 - RNA, 3245 nt, Homo sapiens
  source 1..3245: mol_type = other RNA
tgagctgctgtaccaaaataccacaaactgcatggcttaaaacaacagaaatttattccctcacaatcctggaggccagatgtctgaaatcaagatattggtagggttggttccttctcgagactctgagggagaatctgtgacatgcctgttttcctagcttctagtgacttcctccaattcttagggttctttggctcatagatgcattgctctaatctctgcctccatcttcccatggccttcagctctgtgtgtctatttccccttcttttctaagagctagtcattgaatttagggcccaccctactacaggttgatctcatttccaggtccttgatttcatctgcaaaaactttttccaaataatgtcacacgtggagattcccagtgaatgtatctcctgggggccactattcagcctattacactattcttagaagatgcctagaaggatatggccaatgttatccagaaggcttcatgaaggaggtaatagaagctaacccttcaaagatgaaagttggcgttcattagagggtcacaaggggaggaagggaatgtcaggttcagggaccagccagaccagagctaaggaagtgacatcacatggaacaatttgtgaacagcaagcagtagggcctggctgcaggacagggtgtgaagtgggggagcagtgatcaggagggccagagagatcagcagggatgtgatcttgagaagctgtgtgtgccatgatctggccctattaatccagaagggtctgatggaagcctctgtgattctcttccatggttaaacattttaattgtattatacctcggatattcctaaatatttaaaacactggcatggttgaactagacaacctttaagtagtttgttccaaccatgagatttagatttcatgatttaggttttatgatcttaaactgaaacctgttagttttctaccactagtgagatcatggcctctgcttttctcctgggaagtccctcttataatcactctcttcccatgattaaagggctactctgccttcatgttgctacccgctcccctggaaatggagaatcaagcaaggatgcggttttccttccattactacatccatacaagagtaaatcaagaataaaagtccagttaatgaaaagatcactggtcttaatatacttagcaaaattttaaaggcaattaaaagtatatacatagacaatgatcaaaattctaatgaaaagacccggctctcccctaaaagaagaaaaaatcatgtaatgtatatatgcattccataaaaacatacatggggaaaacttcagaagcctaaaaacaaaacatcagtaaaccaagccacacttagaaaaatgaaagctgatttttattttatcatcaacagccattctttagacatgaacatgcatacgtaatattctacgcacacatcacagcttttaacgttagttaataaaggttaaacacacaacatacatccttacaaaaaaagtcaaaatgcaaacttaaaactttaaacaaaagtattactaatttaaaaaaagtttgtgttgggtaccatttgtacaacacagttaatttaaacattttcattttggttgcacatgaaaaaggcggcagtagaaaataaagtcattgagggtttttaaatagcagaataggcagttttgccatgcaggagaagcaatattaaatattagtttcaaaaaaaatccacatttaaaaatatttagttcaagtcacagaatttttctcagtagagaccccaatgcaatgcataattagctgccttagatggcccgtttgaaaggatgatatcccttcagagtgtaactttactgattttggcacagaaaagaagtcttaagaacatgattaaaaaagagggaagaggaacagaggaaagaaataaaagcaagaataaatgagatagtaattgcaatcactaaaaaactgcattctcagtcattgcagaatactgtcttctgtctacagcaggtgcttattccagaattgttattgcagcatggatttaatttgcttggaggtagtctcatcattcaaatgttttgttgtgtacctgagagcatttagaagaccttccacactattaggaggttggtccttaagaactttgatacaacctttcatatcaattttggaagttttagcaaatgctcccactggatgtacgtggtcatagagtattatgacacccaccattaccctcaagcagaatgacactgtctcttcatttgtaaatctgcttctgtattccggtgtttccagcatgactctgcatacactagccattgtgcttaaacaatctgtggtattttctattggtaaatttttattctctgatacaaattttgttgtggcatcactcaaggttttcagcattggagttgcctcagcataaaacaaagacattcgatttgccaattcattatttacttcattttctccttctgccggtacattgttaatcctcatacgactcaatgttcttctataatagctgaaatcattctgtatggcaggatttgtcatcttgagttcatcaaaccggagtgtgaaatgaagaatttctgcaaactgtttagcaagagcctgctctcgctctagatgctgggtgggagaatatggggtacttgttaaggctcccagaagacctcttaatgctgcttctaacctctgagaaaattcgtaaaatttctttaatttgcctactagtggaacaactgcaccccatgccttctcttgcaacttctcatctgctggatgctggattgcctctcgtatttcgtggccagctcctctgtatgactgcaagtcctccaagatgccttctgcatcttttaatactacattcacctgattataaatttccttctcagactctgtaggctgggcattttcaaaatcaaggaaaaaatttggcccctgctcaaggtctgtgcatgtcaaaactttaagaagattccccatgttaaggtaccttcagccagtgctggtgattctgtccttgtccttctatctggcggcccgggcgggcgaggggagcgcggcgcgggagcgcaggagcctcggagcctccggtgccgccgccgccgccgtttccgggttggcggggctcacgtcaccgccacaggtttgcgagctgcccccgccgcggcggcagcagcagcagcagcagcagcccgggcgagtgccaggcgagaaataact

SEQ ID NO: 18495 - RNA, 3145 nt, Homo sapiens
  source 1..3145: mol_type = other RNA
tgagctgctgtaccaaaataccacaaactgcatggcttaaaacaacagaaatttattccctcacaatcctggaggccagatgtctgaaatcaagatattggtagggttggttccttctcgagactctgagggagaatctgtgacatgcctgttttcctagcttctagtgacttcctccaattcttagggttctttggctcatagatgcattgctctaatctctgcctccatcttcccatggccttcagctctgtgtgtctatttccccttcttttctaagagctagtcattgaatttagggcccaccctactacaggttgatctcatttccaggtccttgatttcatctgcaaaaactttttccaaataatgtcacacgtggagattcccagtgaatgtatctcctgggggccactattcagcctattacactattcttagaagatgcctagaaggatatggccaatgttatccagaaggcttcatgaaggaggtaatagaagctaacccttcaaagatgaaagttggcgttcattagagggtcacaaggggaggaagggaatgtcaggttcagggaccagccagaccagagctaaggaagtgacatcacatggaacaatttgtgaacagcaagcagtagggcctggctgcaggacagggtgtgaagtgggggagcagtgatcaggagggccagagagatcagcagggatgtgatcttgagaagctgtgtgtgccatgatctggccctattaatccagaagggtctgatggaagcctctgtgattctcttccatggttaaacattttaattgtattatacctcggatattcctaaatatttaaaacactggcatggttgaactagacaacctttaagtagtttgttccaaccatgagatttagatttcatgatttaggttttatgatcttaaactgaaacctgttagttttctaccactagtgagatcatggcctctgcttttctcctgggaagtccctcttataatcactctcttcccatgattaaagggctactctgccttcatgttgctacccgctcccctggaaatggagaatcaagcaaggatgcggttttccttccattactacatccatacaagagtaaatcaagaataaaagtccagttaatgaaaagatcactggtcttaatatacttagcaaaattttaaaggcaattaaaagtatatacatagacaatgatcaaaattctaatgaaaagacccggctctcccctaaaagaagaaaaaatcatgtaatgtatatatgcattccataaaaacatacatggggaaaacttcagaagcctaaaaacaaaacatcagtaaaccaagccacacttagaaaaatgaaagctgatttttattttatcatcaacagccattctttagacatgaacatgcatacgtaatattctacgcacacatcacagcttttaacgttagttaataaaggttaaacacacaacatacatccttacaaaaaaagtcaaaatgcaaacttaaaactttaaacaaaagtattactaatttaaaaaaagtttgtgttgggtaccatttgtacaacacagttaatttaaacattttcattttggttgcacatgaaaaaggcggcagtagaaaataaagtcattgagggtttttaaatagcagaataggcagttttgccatgcaggagaagcaatattaaatattagtttcaaaaaaaatccacatttaaaaatatttagttcaagtcacagaatttttctcagtagagaccccaatgcaatgcataattagctgccttagatggcccgtttgaaaggatgatatcccttcagagtgtaactttactgattttggcacagaaaagaagtcttaagaacatgattaaaaaagagggaagaggaacagaggaaagaaataaaagcaagaataaatgagatagtaattgcaatcactaaaaaactgcattctcagtcattgcagaatactgtcttctgtctacagcaggtgcttattccagaattgttattgcagcatggatttaatttgcttggaggtagtctcatcattcaaatgttttgttgtgtacctgagagcatttagaagaccttccacactattaggaggttggtccttaagaactttgatacaacctttcatatcaattttggaagttttagcaaatgctcccactggatgtacgtggtcatagagtattatgacacccaccattaccctcaagcagaatgacactgtctcttcatttgtaaatctgcttctgtattccggtgtttccagcatgactctgcatacactagccattgtgcttaaacaatctgtggtattttctattggtaaatttttattctctgatacaaattttgttgtggcatcactcaaggttttcagcattggagttgcctcagcataaaacaaagacattcgatttgccaattcattatttacttcattttctccttctgccggtacattgttaatcctcatacgactcaatgttcttctataatagctgaaatcattctgtatggcaggatttgtcatcttgagttcatcaaaccggagtgtgaaatgaagaatttctgcaaactgtttagcaagagcctgctctcgctctagatgctgggtgggagaatatggggtacttgttaaggctcccagaagacctcttaatgctgcttctaacctctgagaaaattcgtaaaatttctttaatttgcctactagtggaacaactgcaccccatgccttctcttgcaacttctcatctgctggatgctggattgcctctcgtatttcgtggccagctcctctgtatgactgcaagtcctccaagatgccttctgcatcttttaatactacattcacctgattataaatttccttctcagactctgtaggctgggcattttcaaaatcaaggaaaaaatttggcccctgctcaaggtctgtgcatgtcaaaactttaagaagattccccatgttaaggtaccttcagccagtgctggtgattctgtccttgtccttctatcttcgagaagccgagccgccggcgctcgcacaaaaggaggacgctcgcctcgcgacgcgcctccccccgcgcccagtccccgccgcatcgc

SEQ ID NO: 18496 - RNA, 3491 nt, Homo sapiens
  source 1..3491: mol_type = other RNA
tgagctgctgtaccaaaataccacaaactgcatggcttaaaacaacagaaatttattccctcacaatcctggaggccagatgtctgaaatcaagatattggtagggttggttccttctcgagactctgagggagaatctgtgacatgcctgttttcctagcttctagtgacttcctccaattcttagggttctttggctcatagatgcattgctctaatctctgcctccatcttcccatggccttcagctctgtgtgtctatttccccttcttttctaagagctagtcattgaatttagggcccaccctactacaggttgatctcatttccaggtccttgatttcatctgcaaaaactttttccaaataatgtcacacgtggagattcccagtgaatgtatctcctgggggccactattcagcctattacactattcttagaagatgcctagaaggatatggccaatgttatccagaaggcttcatgaaggaggtaatagaagctaacccttcaaagatgaaagttggcgttcattagagggtcacaaggggaggaagggaatgtcaggttcagggaccagccagaccagagctaaggaagtgacatcacatggaacaatttgtgaacagcaagcagtagggcctggctgcaggacagggtgtgaagtgggggagcagtgatcaggagggccagagagatcagcagggatgtgatcttgagaagctgtgtgtgccatgatctggccctattaatccagaagggtctgatggaagcctctgtgattctcttccatggttaaacattttaattgtattatacctcggatattcctaaatatttaaaacactggcatggttgaactagacaacctttaagtagtttgttccaaccatgagatttagatttcatgatttaggttttatgatcttaaactgaaacctgttagttttctaccactagtgagatcatggcctctgcttttctcctgggaagtccctcttataatcactctcttcccatgattaaagggctactctgccttcatgttgctacccgctcccctggaaatggagaatcaagcaaggatgcggttttccttccattactacatccatacaagagtaaatcaagaataaaagtccagttaatgaaaagatcactggtcttaatatacttagcaaaattttaaaggcaattaaaagtatatacatagacaatgatcaaaattctaatgaaaagacccggctctcccctaaaagaagaaaaaatcatgtaatgtatatatgcattccataaaaacatacatggggaaaacttcagaagcctaaaaacaaaacatcagtaaaccaagccacacttagaaaaatgaaagctgatttttattttatcatcaacagccattctttagacatgaacatgcatacgtaatattctacgcacacatcacagcttttaacgttagttaataaaggttaaacacacaacatacatccttacaaaaaaagtcaaaatgcaaacttaaaactttaaacaaaagtattactaatttaaaaaaagtttgtgttgggtaccatttgtacaacacagttaatttaaacattttcattttggttgcacatgaaaaaggcggcagtagaaaataaagtcattgagggtttttaaatagcagaataggcagttttgccatgcaggagaagcaatattaaatattagtttcaaaaaaaatccacatttaaaaatatttagttcaagtcacagaatttttctcagtagagaccccaatgcaatgcataattagctgccttagatggcccgtttgaaaggatgatatcccttcagagtgtaactttactgattttggcacagaaaagaagtcttaagaacatgattaaaaaagagggaagaggaacagaggaaagaaataaaagcaagaataaatgagatagtaattgcaatcactaaaaaactgcattctcagtcattgcagaatactgtcttctgtctacagcaggtgcttattccagaattgttattgcagcatggatttaatttgcttggaggtagtctcatcattcaaatgttttgttgtgtacctgagagcatttagaagaccttccacactattaggaggttggtccttaagaactttgatacaacctttcatatcaattttggaagttttagcaaatgctcccactggatgtacgtggtcatagagtattatgacacccaccattaccctcaagcagaatgacactgtctcttcatttgtaaatctgcttctgtattccggtgtttccagcatgactctgcatacactagccattgtgcttaaacaatctgtggtattttctattggtaaatttttattctctgatacaaattttgttgtggcatcactcaaggttttcagcattggagttgcctcagcataaaacaaagacattcgatttgccaattcattatttacttcattttctccttctgccggtacattgttaatcctcatacgactcaatgttcttctataatagctgaaatcattctgtatggcaggatttgtcatcttgagttcatcaaaccggagtgtgaaatgaagaatttctgcaaactgtttagcaagagcctgctctcgctctagatgctgggtgggagaatatggggtacttgttaaggctcccagaagacctcttaatgctgcttctaacctctgagaaaattcgtaaaatttctttaatttgcctactagtggaacaactgcaccccatgccttctcttgcaacttctcatctgctggatgctggattgcctctcgtatttcgtggccagctcctctgtatgactgcaagtcctccaagatgccttctgcatcttttaatactacattcacctgattataaatttccttctcagactctgtaggctgggcattttcaaaatcaaggaaaaaatttggcccctgctcaaggtctgtgcatgtcaaaactttaagaagattccccatgttaaggtactgccaagtaaacaggccttgtggcagtgaaaggataaactgtccatcattctttcttctcctcggagatttcacaggaaaaggagaaagcgcaggaaacaggaggccttcagccagtgctggtgattctgtccttgtccttctatccttggattggcgttccctctttcctagttcacttgttccagtccttcaacttctgtttcttgctaacaggtgtgcaaatgaattaccaactgggtaaccttgaatgagttaatcaaattccaggcctcagtttcttctcctggcggcccgggcgggcgaggggagcgcggcgcgggagcgcaggagcctcggagcctccggtgccgccgccgccgccgtttccgggttggcggggctcacgtcaccgccacaggtttgcgagctgcccccgccgcggcggcagcagcagcagcagcagcagcccgggcgagtgccaggcgagaaataact

SEQ ID NO: 18497 - RNA, 3391 nt, Homo sapiens
  source 1..3391: mol_type = other RNA
tgagctgctgtaccaaaataccacaaactgcatggcttaaaacaacagaaatttattccctcacaatcctggaggccagatgtctgaaatcaagatattggtagggttggttccttctcgagactctgagggagaatctgtgacatgcctgttttcctagcttctagtgacttcctccaattcttagggttctttggctcatagatgcattgctctaatctctgcctccatcttcccatggccttcagctctgtgtgtctatttccccttcttttctaagagctagtcattgaatttagggcccaccctactacaggttgatctcatttccaggtccttgatttcatctgcaaaaactttttccaaataatgtcacacgtggagattcccagtgaatgtatctcctgggggccactattcagcctattacactattcttagaagatgcctagaaggatatggccaatgttatccagaaggcttcatgaaggaggtaatagaagctaacccttcaaagatgaaagttggcgttcattagagggtcacaaggggaggaagggaatgtcaggttcagggaccagccagaccagagctaaggaagtgacatcacatggaacaatttgtgaacagcaagcagtagggcctggctgcaggacagggtgtgaagtgggggagcagtgatcaggagggccagagagatcagcagggatgtgatcttgagaagctgtgtgtgccatgatctggccctattaatccagaagggtctgatggaagcctctgtgattctcttccatggttaaacattttaattgtattatacctcggatattcctaaatatttaaaacactggcatggttgaactagacaacctttaagtagtttgttccaaccatgagatttagatttcatgatttaggttttatgatcttaaactgaaacctgttagttttctaccactagtgagatcatggcctctgcttttctcctgggaagtccctcttataatcactctcttcccatgattaaagggctactctgccttcatgttgctacccgctcccctggaaatggagaatcaagcaaggatgcggttttccttccattactacatccatacaagagtaaatcaagaataaaagtccagttaatgaaaagatcactggtcttaatatacttagcaaaattttaaaggcaattaaaagtatatacatagacaatgatcaaaattctaatgaaaagacccggctctcccctaaaagaagaaaaaatcatgtaatgtatatatgcattccataaaaacatacatggggaaaacttcagaagcctaaaaacaaaacatcagtaaaccaagccacacttagaaaaatgaaagctgatttttattttatcatcaacagccattctttagacatgaacatgcatacgtaatattctacgcacacatcacagcttttaacgttagttaataaaggttaaacacacaacatacatccttacaaaaaaagtcaaaatgcaaacttaaaactttaaacaaaagtattactaatttaaaaaaagtttgtgttgggtaccatttgtacaacacagttaatttaaacattttcattttggttgcacatgaaaaaggcggcagtagaaaataaagtcattgagggtttttaaatagcagaataggcagttttgccatgcaggagaagcaatattaaatattagtttcaaaaaaaatccacatttaaaaatatttagttcaagtcacagaatttttctcagtagagaccccaatgcaatgcataattagctgccttagatggcccgtttgaaaggatgatatcccttcagagtgtaactttactgattttggcacagaaaagaagtcttaagaacatgattaaaaaagagggaagaggaacagaggaaagaaataaaagcaagaataaatgagatagtaattgcaatcactaaaaaactgcattctcagtcattgcagaatactgtcttctgtctacagcaggtgcttattccagaattgttattgcagcatggatttaatttgcttggaggtagtctcatcattcaaatgttttgttgtgtacctgagagcatttagaagaccttccacactattaggaggttggtccttaagaactttgatacaacctttcatatcaattttggaagttttagcaaatgctcccactggatgtacgtggtcatagagtattatgacacccaccattaccctcaagcagaatgacactgtctcttcatttgtaaatctgcttctgtattccggtgtttccagcatgactctgcatacactagccattgtgcttaaacaatctgtggtattttctattggtaaatttttattctctgatacaaattttgttgtggcatcactcaaggttttcagcattggagttgcctcagcataaaacaaagacattcgatttgccaattcattatttacttcattttctccttctgccggtacattgttaatcctcatacgactcaatgttcttctataatagctgaaatcattctgtatggcaggatttgtcatcttgagttcatcaaaccggagtgtgaaatgaagaatttctgcaaactgtttagcaagagcctgctctcgctctagatgctgggtgggagaatatggggtacttgttaaggctcccagaagacctcttaatgctgcttctaacctctgagaaaattcgtaaaatttctttaatttgcctactagtggaacaactgcaccccatgccttctcttgcaacttctcatctgctggatgctggattgcctctcgtatttcgtggccagctcctctgtatgactgcaagtcctccaagatgccttctgcatcttttaatactacattcacctgattataaatttccttctcagactctgtaggctgggcattttcaaaatcaaggaaaaaatttggcccctgctcaaggtctgtgcatgtcaaaactttaagaagattccccatgttaaggtactgccaagtaaacaggccttgtggcagtgaaaggataaactgtccatcattctttcttctcctcggagatttcacaggaaaaggagaaagcgcaggaaacaggaggccttcagccagtgctggtgattctgtccttgtccttctatccttggattggcgttccctctttcctagttcacttgttccagtccttcaacttctgtttcttgctaacaggtgtgcaaatgaattaccaactgggtaaccttgaatgagttaatcaaattccaggcctcagtttcttctccttcgagaagccgagccgccggcgctcgcacaaaaggaggacgctcgcctcgcgacgcgcctccccccgcgcccagtccccgccgcatcgc

SEQ ID NO: 18498 - RNA, 3611 nt, Homo sapiens
  source 1..3611: mol_type = other RNA
tgagctgctgtaccaaaataccacaaactgcatggcttaaaacaacagaaatttattccctcacaatcctggaggccagatgtctgaaatcaagatattggtagggttggttccttctcgagactctgagggagaatctgtgacatgcctgttttcctagcttctagtgacttcctccaattcttagggttctttggctcatagatgcattgctctaatctctgcctccatcttcccatggccttcagctctgtgtgtctatttccccttcttttctaagagctagtcattgaatttagggcccaccctactacaggttgatctcatttccaggtccttgatttcatctgcaaaaactttttccaaataatgtcacacgtggagattcccagtgaatgtatctcctgggggccactattcagcctattacactattcttagaagatgcctagaaggatatggccaatgttatccagaaggcttcatgaaggaggtaatagaagctaacccttcaaagatgaaagttggcgttcattagagggtcacaaggggaggaagggaatgtcaggttcagggaccagccagaccagagctaaggaagtgacatcacatggaacaatttgtgaacagcaagcagtagggcctggctgcaggacagggtgtgaagtgggggagcagtgatcaggagggccagagagatcagcagggatgtgatcttgagaagctgtgtgtgccatgatctggccctattaatccagaagggtctgatggaagcctctgtgattctcttccatggttaaacattttaattgtattatacctcggatattcctaaatatttaaaacactggcatggttgaactagacaacctttaagtagtttgttccaaccatgagatttagatttcatgatttaggttttatgatcttaaactgaaacctgttagttttctaccactagtgagatcatggcctctgcttttctcctgggaagtccctcttataatcactctcttcccatgattaaagggctactctgccttcatgttgctacccgctcccctggaaatggagaatcaagcaaggatgcggttttccttccattactacatccatacaagagtaaatcaagaataaaagtccagttaatgaaaagatcactggtcttaatatacttagcaaaattttaaaggcaattaaaagtatatacatagacaatgatcaaaattctaatgaaaagacccggctctcccctaaaagaagaaaaaatcatgtaatgtatatatgcattccataaaaacatacatggggaaaacttcagaagcctaaaaacaaaacatcagtaaaccaagccacacttagaaaaatgaaagctgatttttattttatcatcaacagccattctttagacatgaacatgcatacgtaatattctacgcacacatcacagcttttaacgttagttaataaaggttaaacacacaacatacatccttacaaaaaaagtcaaaatgcaaacttaaaactttaaacaaaagtattactaatttaaaaaaagtttgtgttgggtaccatttgtacaacacagttaatttaaacattttcattttggttgcacatgaaaaaggcggcagtagaaaataaagtcattgagggtttttaaatagcagaataggcagttttgccatgcaggagaagcaatattaaatattagtttcaaaaaaaatccacatttaaaaatatttagttcaagtcacagaatttttctcagtagagaccccaatgcaatgcataattagctgccttagatggcccgtttgaaaggatgatatcccttcagagtgtaactttactgattttggcacagaaaagaagtcttaagaacatgattaaaaaagagggaagaggaacagaggaaagaaataaaagcaagaataaatgagatagtaattgcaatcactaaaaaactgcattctcagtcattgcagaatactgtcttctgtctacagcaggtgcttattccagaattgttattgcagcatggatttaatttgcttggaggtagtctcatcattcaaatgttttgttgtgtacctgagagcatttagaagaccttccacactattaggaggttggtccttaagaactttgatacaacctttcatatcaattttggaagttttagcaaatgctcccactggatgtacgtggtcatagagtattatgacacccaccattaccctcaagcagaatgacactgtctcttcatttgtaaatctgcttctgtattccggtgtttccagcatgactctgcatacactagccattgtgcttaaacaatctgtggtattttctattggtaaatttttattctctgatacaaattttgttgtggcatcactcaaggttttcagcattggagttgcctcagcataaaacaaagacattcgatttgccaattcattatttacttcattttctccttctgccggtacattgttaatcctcatacgactcaatgttcttctataatagctgaaatcattctgtatggcaggatttgtcatcttgagttcatcaaaccggagtgtgaaatgaagaatttctgcaaactgtttagcaagagcctgctctcgctctagatgctgggtgggagaatatggggtacttgttaaggctcccagaagacctcttaatgctgcttctaacctctgagaaaattcgtaaaatttctttaatttgcctactagtggaacaactgcaccccatgccttctcttgcaacttctcatctgctggatgctggattgcctctcgtatttcgtggccagctcctctgtatgactgcaagtcctccaagatgccttctgcatcttttaatactacattcacctgattataaatttccttctcagactctgtaggctgggcattttcaaaatcaaggaaaaaatttggcccctgctcaaggtctgtgcatgtcaaaactttaagaagattccccatgttaaggtactttcaaagtccaagaaaaaatgtgctgcattgtggtctatgtccctggttagcaccttaatgagattacccatgccagcaaacctccccagagtgagagtctctggtgcctcttccagtcaccaaacagcagcaaaaaagcaaggaacttaaggacctactgccaagtaaacaggccttgtggcagtgaaaggataaactgtccatcattctttcttctcctcggagatttcacaggaaaaggagaaagcgcaggaaacaggaggccttcagccagtgctggtgattctgtccttgtccttctatccttggattggcgttccctctttcctagttcacttgttccagtccttcaacttctgtttcttgctaacaggtgtgcaaatgaattaccctccgctcgagcctccaggcgctctcagtcccgctcctgcgccctcctggagccgcagaggcggctcctcagcggcgctagggggagccccgggtccggagcgggggagcggcggcagccggaccgggagcccctcaacacctgcccctgtggcagagccgcgacaagccaggcggcagctccgagcggggagggcaagtgac

SEQ ID NO: 18499 - RNA, 3381 nt, Homo sapiens
  source 1..3381: mol_type = other RNA
tgagctgctgtaccaaaataccacaaactgcatggcttaaaacaacagaaatttattccctcacaatcctggaggccagatgtctgaaatcaagatattggtagggttggttccttctcgagactctgagggagaatctgtgacatgcctgttttcctagcttctagtgacttcctccaattcttagggttctttggctcatagatgcattgctctaatctctgcctccatcttcccatggccttcagctctgtgtgtctatttccccttcttttctaagagctagtcattgaatttagggcccaccctactacaggttgatctcatttccaggtccttgatttcatctgcaaaaactttttccaaataatgtcacacgtggagattcccagtgaatgtatctcctgggggccactattcagcctattacactattcttagaagatgcctagaaggatatggccaatgttatccagaaggcttcatgaaggaggtaatagaagctaacccttcaaagatgaaagttggcgttcattagagggtcacaaggggaggaagggaatgtcaggttcagggaccagccagaccagagctaaggaagtgacatcacatggaacaatttgtgaacagcaagcagtagggcctggctgcaggacagggtgtgaagtgggggagcagtgatcaggagggccagagagatcagcagggatgtgatcttgagaagctgtgtgtgccatgatctggccctattaatccagaagggtctgatggaagcctctgtgattctcttccatggttaaacattttaattgtattatacctcggatattcctaaatatttaaaacactggcatggttgaactagacaacctttaagtagtttgttccaaccatgagatttagatttcatgatttaggttttatgatcttaaactgaaacctgttagttttctaccactagtgagatcatggcctctgcttttctcctgggaagtccctcttataatcactctcttcccatgattaaagggctactctgccttcatgttgctacccgctcccctggaaatggagaatcaagcaaggatgcggttttccttccattactacatccatacaagagtaaatcaagaataaaagtccagttaatgaaaagatcactggtcttaatatacttagcaaaattttaaaggcaattaaaagtatatacatagacaatgatcaaaattctaatgaaaagacccggctctcccctaaaagaagaaaaaatcatgtaatgtatatatgcattccataaaaacatacatggggaaaacttcagaagcctaaaaacaaaacatcagtaaaccaagccacacttagaaaaatgaaagctgatttttattttatcatcaacagccattctttagacatgaacatgcatacgtaatattctacgcacacatcacagcttttaacgttagttaataaaggttaaacacacaacatacatccttacaaaaaaagtcaaaatgcaaacttaaaactttaaacaaaagtattactaatttaaaaaaagtttgtgttgggtaccatttgtacaacacagttaatttaaacattttcattttggttgcacatgaaaaaggcggcagtagaaaataaagtcattgagggtttttaaatagcagaataggcagttttgccatgcaggagaagcaatattaaatattagtttcaaaaaaaatccacatttaaaaatatttagttcaagtcacagaatttttctcagtagagaccccaatgcaatgcataattagctgccttagatggcccgtttgaaaggatgatatcccttcagagtgtaactttactgattttggcacagaaaagaagtcttaagaacatgattaaaaaagagggaagaggaacagaggaaagaaataaaagcaagaataaatgagatagtaattgcaatcactaaaaaactgcattctcagtcattgcagaatactgtcttctgtctacagcaggtgcttattccagaattgttattgcagcatggatttaatttgcttggaggtagtctcatcattcaaatgttttgttgtgtacctgagagcatttagaagaccttccacactattaggaggttggtccttaagaactttgatacaacctttcatatcaattttggaagttttagcaaatgctcccactggatgtacgtggtcatagagtattatgacacccaccattaccctcaagcagaatgacactgtctcttcatttgtaaatctgcttctgtattccggtgtttccagcatgactctgcatacactagccattgtgcttaaacaatctgtggtattttctattggtaaatttttattctctgatacaaattttgttgtggcatcactcaaggttttcagcattggagttgcctcagcataaaacaaagacattcgatttgccaattcattatttacttcattttctccttctgccggtacattgttaatcctcatacgactcaatgttcttctataatagctgaaatcattctgtatggcaggatttgtcatcttgagttcatcaaaccggagtgtgaaatgaagaatttctgcaaactgtttagcaagagcctgctctcgctctagatgctgggtgggagaatatggggtacttgttaaggctcccagaagacctcttaatgctgcttctaacctctgagaaaattcgtaaaatttctttaatttgcctactagtggaacaactgcaccccatgccttctcttgcaacttctcatctgctggatgctggattgcctctcgtatttcgtggccagctcctctgtatgactgcaagtcctccaagatgccttctgcatcttttaatactacattcacctgattataaatttccttctcagactctgtaggctgggcattttcaaaatcaaggaaaaaatttggcccctgctcaaggtctgtgcatgtcaaaactttaagaagattccccatgttaaggtactttcaaagtccaagaaaaaatgtgctgcattgtggtctatgtccctggttagcaccttaatgagattacccatgccagcaaaccttcagccagtgctggtgattctgtccttgtccttctatcaactgggtaaccttgaatgagttaatcaaattccaggcctcagtttcttctcctggcggcccgggcgggcgaggggagcgcggcgcgggagcgcaggagcctcggagcctccggtgccgccgccgccgccgtttccgggttggcggggctcacgtcaccgccacaggtttgcgagctgcccccgccgcggcggcagcagcagcagcagcagcagcccgggcgagtgccaggcgagaaataact

SEQ ID NO: 18500 - RNA, 3341 nt, Homo sapiens
  source 1..3341: mol_type = other RNA
tgagctgctgtaccaaaataccacaaactgcatggcttaaaacaacagaaatttattccctcacaatcctggaggccagatgtctgaaatcaagatattggtagggttggttccttctcgagactctgagggagaatctgtgacatgcctgttttcctagcttctagtgacttcctccaattcttagggttctttggctcatagatgcattgctctaatctctgcctccatcttcccatggccttcagctctgtgtgtctatttccccttcttttctaagagctagtcattgaatttagggcccaccctactacaggttgatctcatttccaggtccttgatttcatctgcaaaaactttttccaaataatgtcacacgtggagattcccagtgaatgtatctcctgggggccactattcagcctattacactattcttagaagatgcctagaaggatatggccaatgttatccagaaggcttcatgaaggaggtaatagaagctaacccttcaaagatgaaagttggcgttcattagagggtcacaaggggaggaagggaatgtcaggttcagggaccagccagaccagagctaaggaagtgacatcacatggaacaatttgtgaacagcaagcagtagggcctggctgcaggacagggtgtgaagtgggggagcagtgatcaggagggccagagagatcagcagggatgtgatcttgagaagctgtgtgtgccatgatctggccctattaatccagaagggtctgatggaagcctctgtgattctcttccatggttaaacattttaattgtattatacctcggatattcctaaatatttaaaacactggcatggttgaactagacaacctttaagtagtttgttccaaccatgagatttagatttcatgatttaggttttatgatcttaaactgaaacctgttagttttctaccactagtgagatcatggcctctgcttttctcctgggaagtccctcttataatcactctcttcccatgattaaagggctactctgccttcatgttgctacccgctcccctggaaatggagaatcaagcaaggatgcggttttccttccattactacatccatacaagagtaaatcaagaataaaagtccagttaatgaaaagatcactggtcttaatatacttagcaaaattttaaaggcaattaaaagtatatacatagacaatgatcaaaattctaatgaaaagacccggctctcccctaaaagaagaaaaaatcatgtaatgtatatatgcattccataaaaacatacatggggaaaacttcagaagcctaaaaacaaaacatcagtaaaccaagccacacttagaaaaatgaaagctgatttttattttatcatcaacagccattctttagacatgaacatgcatacgtaatattctacgcacacatcacagcttttaacgttagttaataaaggttaaacacacaacatacatccttacaaaaaaagtcaaaatgcaaacttaaaactttaaacaaaagtattactaatttaaaaaaagtttgtgttgggtaccatttgtacaacacagttaatttaaacattttcattttggttgcacatgaaaaaggcggcagtagaaaataaagtcattgagggtttttaaatagcagaataggcagttttgccatgcaggagaagcaatattaaatattagtttcaaaaaaaatccacatttaaaaatatttagttcaagtcacagaatttttctcagtagagaccccaatgcaatgcataattagctgccttagatggcccgtttgaaaggatgatatcccttcagagtgtaactttactgattttggcacagaaaagaagtcttaagaacatgattaaaaaagagggaagaggaacagaggaaagaaataaaagcaagaataaatgagatagtaattgcaatcactaaaaaactgcattctcagtcattgcagaatactgtcttctgtctacagcaggtgcttattccagaattgttattgcagcatggatttaatttgcttggaggtagtctcatcattcaaatgttttgttgtgtacctgagagcatttagaagaccttccacactattaggaggttggtccttaagaactttgatacaacctttcatatcaattttggaagttttagcaaatgctcccactggatgtacgtggtcatagagtattatgacacccaccattaccctcaagcagaatgacactgtctcttcatttgtaaatctgcttctgtattccggtgtttccagcatgactctgcatacactagccattgtgcttaaacaatctgtggtattttctattggtaaatttttattctctgatacaaattttgttgtggcatcactcaaggttttcagcattggagttgcctcagcataaaacaaagacattcgatttgccaattcattatttacttcattttctccttctgccggtacattgttaatcctcatacgactcaatgttcttctataatagctgaaatcattctgtatggcaggatttgtcatcttgagttcatcaaaccggagtgtgaaatgaagaatttctgcaaactgtttagcaagagcctgctctcgctctagatgctgggtgggagaatatggggtacttgttaaggctcccagaagacctcttaatgctgcttctaacctctgagaaaattcgtaaaatttctttaatttgcctactagtggaacaactgcaccccatgccttctcttgcaacttctcatctgctggatgctggattgcctctcgtatttcgtggccagctcctctgtatgactgcaagtcctccaagatgccttctgcatcttttaatactacattcacctgattataaatttccttctcagactctgtaggctgggcattttcaaaatcaaggaaaaaatttggcccctgctcaaggtctgtgcatgtcaaaactttaagaagattccccatgttaaggtactttcaaagtccaagaaaaaatgtgctgcattgtggtctatgtccctggttagcaccttaatgagattacccatgccagcaaaccttcagccagtgctggtgattctgtccttgtccttctatcctccgctcgagcctccaggcgctctcagtcccgctcctgcgccctcctggagccgcagaggcggctcctcagcggcgctagggggagccccgggtccggagcgggggagcggcggcagccggaccgggagcccctcaacacctgcccctgtggcagagccgcgacaagccaggcggcagctccgagcggggagggcaagtgac

SEQ ID NO: 18501 - RNA, 3468 nt, Homo sapiens
  source 1..3468: mol_type = other RNA
tgagctgctgtaccaaaataccacaaactgcatggcttaaaacaacagaaatttattccctcacaatcctggaggccagatgtctgaaatcaagatattggtagggttggttccttctcgagactctgagggagaatctgtgacatgcctgttttcctagcttctagtgacttcctccaattcttagggttctttggctcatagatgcattgctctaatctctgcctccatcttcccatggccttcagctctgtgtgtctatttccccttcttttctaagagctagtcattgaatttagggcccaccctactacaggttgatctcatttccaggtccttgatttcatctgcaaaaactttttccaaataatgtcacacgtggagattcccagtgaatgtatctcctgggggccactattcagcctattacactattcttagaagatgcctagaaggatatggccaatgttatccagaaggcttcatgaaggaggtaatagaagctaacccttcaaagatgaaagttggcgttcattagagggtcacaaggggaggaagggaatgtcaggttcagggaccagccagaccagagctaaggaagtgacatcacatggaacaatttgtgaacagcaagcagtagggcctggctgcaggacagggtgtgaagtgggggagcagtgatcaggagggccagagagatcagcagggatgtgatcttgagaagctgtgtgtgccatgatctggccctattaatccagaagggtctgatggaagcctctgtgattctcttccatggttaaacattttaattgtattatacctcggatattcctaaatatttaaaacactggcatggttgaactagacaacctttaagtagtttgttccaaccatgagatttagatttcatgatttaggttttatgatcttaaactgaaacctgttagttttctaccactagtgagatcatggcctctgcttttctcctgggaagtccctcttataatcactctcttcccatgattaaagggctactctgccttcatgttgctacccgctcccctggaaatggagaatcaagcaaggatgcggttttccttccattactacatccatacaagagtaaatcaagaataaaagtccagttaatgaaaagatcactggtcttaatatacttagcaaaattttaaaggcaattaaaagtatatacatagacaatgatcaaaattctaatgaaaagacccggctctcccctaaaagaagaaaaaatcatgtaatgtatatatgcattccataaaaacatacatggggaaaacttcagaagcctaaaaacaaaacatcagtaaaccaagccacacttagaaaaatgaaagctgatttttattttatcatcaacagccattctttagacatgaacatgcatacgtaatattctacgcacacatcacagcttttaacgttagttaataaaggttaaacacacaacatacatccttacaaaaaaagtcaaaatgcaaacttaaaactttaaacaaaagtattactaatttaaaaaaagtttgtgttgggtaccatttgtacaacacagttaatttaaacattttcattttggttgcacatgaaaaaggcggcagtagaaaataaagtcattgagggtttttaaatagcagaataggcagttttgccatgcaggagaagcaatattaaatattagtttcaaaaaaaatccacatttaaaaatatttagttcaagtcacagaatttttctcagtagagaccccaatgcaatgcataattagctgccttagatggcccgtttgaaaggatgatatcccttcagagtgtaactttactgattttggcacagaaaagaagtcttaagaacatgattaaaaaagagggaagaggaacagaggaaagaaataaaagcaagaataaatgagatagtaattgcaatcactaaaaaactgcattctcagtcattgcagaatactgtcttctgtctacagcaggtgcttattccagaattgttattgcagcatggatttaatttgcttggaggtagtctcatcattcaaatgttttgttgtgtacctgagagcatttagaagaccttccacactattaggaggttggtccttaagaactttgatacaacctttcatatcaattttggaagttttagcaaatgctcccactggatgtacgtggtcatagagtattatgacacccaccattaccctcaagcagaatgacactgtctcttcatttgtaaatctgcttctgtattccggtgtttccagcatgactctgcatacactagccattgtgcttaaacaatctgtggtattttctattggtaaatttttattctctgatacaaattttgttgtggcatcactcaaggttttcagcattggagttgcctcagcataaaacaaagacattcgatttgccaattcattatttacttcattttctccttctgccggtacattgttaatcctcatacgactcaatgttcttctataatagctgaaatcattctgtatggcaggatttgtcatcttgagttcatcaaaccggagtgtgaaatgaagaatttctgcaaactgtttagcaagagcctgctctcgctctagatgctgggtgggagaatatggggtacttgttaaggctcccagaagacctcttaatgctgcttctaacctctgagaaaattcgtaaaatttctttaatttgcctactagtggaacaactgcaccccatgccttctcttgcaacttctcatctgctggatgctggattgcctctcgtatttcgtggccagctcctctgtatgactgcaagtcctccaagatgccttctgcatcttttaatactacattcacctgattataaatttccttctcagactctgtaggctgggcattttcaaaatcaaggaaaaaatttggcccctgctcaaggtctgtgcatgtcaaaactttaagaagattccccatgttaaggtactttcaaagtccaagaaaaaatgtgctgcattgtggtctatgtccctggttagcaccttaatgagattacccatgccagcaaaccttcagccagtgctggtgattctgtccttgtccttctatccttggattggcgttccctctttcctagttcacttgttccagtccttcaacttctgtttcttgctaacaggtgtgcaaatgaattaccaactgggtaaccttgaatgagttaatcaaattccaggcctcagtttcttctcctggcggcccgggcgggcgaggggagcgcggcgcgggagcgcaggagcctcggagcctccggtgccgccgccgccgccgtttccgggttggcggggctcacgtcaccgccacaggtttgcgagctgcccccgccgcggcggcagcagcagcagcagcagcagcccgggcgagtgccaggcgagaaataact

SEQ ID NO: 18502 - RNA, 3428 nt, Homo sapiens
  source 1..3428: mol_type = other RNA
tgagctgctgtaccaaaataccacaaactgcatggcttaaaacaacagaaatttattccctcacaatcctggaggccagatgtctgaaatcaagatattggtagggttggttccttctcgagactctgagggagaatctgtgacatgcctgttttcctagcttctagtgacttcctccaattcttagggttctttggctcatagatgcattgctctaatctctgcctccatcttcccatggccttcagctctgtgtgtctatttccccttcttttctaagagctagtcattgaatttagggcccaccctactacaggttgatctcatttccaggtccttgatttcatctgcaaaaactttttccaaataatgtcacacgtggagattcccagtgaatgtatctcctgggggccactattcagcctattacactattcttagaagatgcctagaaggatatggccaatgttatccagaaggcttcatgaaggaggtaatagaagctaacccttcaaagatgaaagttggcgttcattagagggtcacaaggggaggaagggaatgtcaggttcagggaccagccagaccagagctaaggaagtgacatcacatggaacaatttgtgaacagcaagcagtagggcctggctgcaggacagggtgtgaagtgggggagcagtgatcaggagggccagagagatcagcagggatgtgatcttgagaagctgtgtgtgccatgatctggccctattaatccagaagggtctgatggaagcctctgtgattctcttccatggttaaacattttaattgtattatacctcggatattcctaaatatttaaaacactggcatggttgaactagacaacctttaagtagtttgttccaaccatgagatttagatttcatgatttaggttttatgatcttaaactgaaacctgttagttttctaccactagtgagatcatggcctctgcttttctcctgggaagtccctcttataatcactctcttcccatgattaaagggctactctgccttcatgttgctacccgctcccctggaaatggagaatcaagcaaggatgcggttttccttccattactacatccatacaagagtaaatcaagaataaaagtccagttaatgaaaagatcactggtcttaatatacttagcaaaattttaaaggcaattaaaagtatatacatagacaatgatcaaaattctaatgaaaagacccggctctcccctaaaagaagaaaaaatcatgtaatgtatatatgcattccataaaaacatacatggggaaaacttcagaagcctaaaaacaaaacatcagtaaaccaagccacacttagaaaaatgaaagctgatttttattttatcatcaacagccattctttagacatgaacatgcatacgtaatattctacgcacacatcacagcttttaacgttagttaataaaggttaaacacacaacatacatccttacaaaaaaagtcaaaatgcaaacttaaaactttaaacaaaagtattactaatttaaaaaaagtttgtgttgggtaccatttgtacaacacagttaatttaaacattttcattttggttgcacatgaaaaaggcggcagtagaaaataaagtcattgagggtttttaaatagcagaataggcagttttgccatgcaggagaagcaatattaaatattagtttcaaaaaaaatccacatttaaaaatatttagttcaagtcacagaatttttctcagtagagaccccaatgcaatgcataattagctgccttagatggcccgtttgaaaggatgatatcccttcagagtgtaactttactgattttggcacagaaaagaagtcttaagaacatgattaaaaaagagggaagaggaacagaggaaagaaataaaagcaagaataaatgagatagtaattgcaatcactaaaaaactgcattctcagtcattgcagaatactgtcttctgtctacagcaggtgcttattccagaattgttattgcagcatggatttaatttgcttggaggtagtctcatcattcaaatgttttgttgtgtacctgagagcatttagaagaccttccacactattaggaggttggtccttaagaactttgatacaacctttcatatcaattttggaagttttagcaaatgctcccactggatgtacgtggtcatagagtattatgacacccaccattaccctcaagcagaatgacactgtctcttcatttgtaaatctgcttctgtattccggtgtttccagcatgactctgcatacactagccattgtgcttaaacaatctgtggtattttctattggtaaatttttattctctgatacaaattttgttgtggcatcactcaaggttttcagcattggagttgcctcagcataaaacaaagacattcgatttgccaattcattatttacttcattttctccttctgccggtacattgttaatcctcatacgactcaatgttcttctataatagctgaaatcattctgtatggcaggatttgtcatcttgagttcatcaaaccggagtgtgaaatgaagaatttctgcaaactgtttagcaagagcctgctctcgctctagatgctgggtgggagaatatggggtacttgttaaggctcccagaagacctcttaatgctgcttctaacctctgagaaaattcgtaaaatttctttaatttgcctactagtggaacaactgcaccccatgccttctcttgcaacttctcatctgctggatgctggattgcctctcgtatttcgtggccagctcctctgtatgactgcaagtcctccaagatgccttctgcatcttttaatactacattcacctgattataaatttccttctcagactctgtaggctgggcattttcaaaatcaaggaaaaaatttggcccctgctcaaggtctgtgcatgtcaaaactttaagaagattccccatgttaaggtactttcaaagtccaagaaaaaatgtgctgcattgtggtctatgtccctggttagcaccttaatgagattacccatgccagcaaaccttcagccagtgctggtgattctgtccttgtccttctatccttggattggcgttccctctttcctagttcacttgttccagtccttcaacttctgtttcttgctaacaggtgtgcaaatgaattaccctccgctcgagcctccaggcgctctcagtcccgctcctgcgccctcctggagccgcagaggcggctcctcagcggcgctagggggagccccgggtccggagcgggggagcggcggcagccggaccgggagcccctcaacacctgcccctgtggcagagccgcgacaagccaggcggcagctccgagcggggagggcaagtgac

SEQ ID NO: 18503 - RNA, 3528 nt, Homo sapiens
  source 1..3528: mol_type = other RNA
tgagctgctgtaccaaaataccacaaactgcatggcttaaaacaacagaaatttattccctcacaatcctggaggccagatgtctgaaatcaagatattggtagggttggttccttctcgagactctgagggagaatctgtgacatgcctgttttcctagcttctagtgacttcctccaattcttagggttctttggctcatagatgcattgctctaatctctgcctccatcttcccatggccttcagctctgtgtgtctatttccccttcttttctaagagctagtcattgaatttagggcccaccctactacaggttgatctcatttccaggtccttgatttcatctgcaaaaactttttccaaataatgtcacacgtggagattcccagtgaatgtatctcctgggggccactattcagcctattacactattcttagaagatgcctagaaggatatggccaatgttatccagaaggcttcatgaaggaggtaatagaagctaacccttcaaagatgaaagttggcgttcattagagggtcacaaggggaggaagggaatgtcaggttcagggaccagccagaccagagctaaggaagtgacatcacatggaacaatttgtgaacagcaagcagtagggcctggctgcaggacagggtgtgaagtgggggagcagtgatcaggagggccagagagatcagcagggatgtgatcttgagaagctgtgtgtgccatgatctggccctattaatccagaagggtctgatggaagcctctgtgattctcttccatggttaaacattttaattgtattatacctcggatattcctaaatatttaaaacactggcatggttgaactagacaacctttaagtagtttgttccaaccatgagatttagatttcatgatttaggttttatgatcttaaactgaaacctgttagttttctaccactagtgagatcatggcctctgcttttctcctgggaagtccctcttataatcactctcttcccatgattaaagggctactctgccttcatgttgctacccgctcccctggaaatggagaatcaagcaaggatgcggttttccttccattactacatccatacaagagtaaatcaagaataaaagtccagttaatgaaaagatcactggtcttaatatacttagcaaaattttaaaggcaattaaaagtatatacatagacaatgatcaaaattctaatgaaaagacccggctctcccctaaaagaagaaaaaatcatgtaatgtatatatgcattccataaaaacatacatggggaaaacttcagaagcctaaaaacaaaacatcagtaaaccaagccacacttagaaaaatgaaagctgatttttattttatcatcaacagccattctttagacatgaacatgcatacgtaatattctacgcacacatcacagcttttaacgttagttaataaaggttaaacacacaacatacatccttacaaaaaaagtcaaaatgcaaacttaaaactttaaacaaaagtattactaatttaaaaaaagtttgtgttgggtaccatttgtacaacacagttaatttaaacattttcattttggttgcacatgaaaaaggcggcagtagaaaataaagtcattgagggtttttaaatagcagaataggcagttttgccatgcaggagaagcaatattaaatattagtttcaaaaaaaatccacatttaaaaatatttagttcaagtcacagaatttttctcagtagagaccccaatgcaatgcataattagctgccttagatggcccgtttgaaaggatgatatcccttcagagtgtaactttactgattttggcacagaaaagaagtcttaagaacatgattaaaaaagagggaagaggaacagaggaaagaaataaaagcaagaataaatgagatagtaattgcaatcactaaaaaactgcattctcagtcattgcagaatactgtcttctgtctacagcaggtgcttattccagaattgttattgcagcatggatttaatttgcttggaggtagtctcatcattcaaatgttttgttgtgtacctgagagcatttagaagaccttccacactattaggaggttggtccttaagaactttgatacaacctttcatatcaattttggaagttttagcaaatgctcccactggatgtacgtggtcatagagtattatgacacccaccattaccctcaagcagaatgacactgtctcttcatttgtaaatctgcttctgtattccggtgtttccagcatgactctgcatacactagccattgtgcttaaacaatctgtggtattttctattggtaaatttttattctctgatacaaattttgttgtggcatcactcaaggttttcagcattggagttgcctcagcataaaacaaagacattcgatttgccaattcattatttacttcattttctccttctgccggtacattgttaatcctcatacgactcaatgttcttctataatagctgaaatcattctgtatggcaggatttgtcatcttgagttcatcaaaccggagtgtgaaatgaagaatttctgcaaactgtttagcaagagcctgctctcgctctagatgctgggtgggagaatatggggtacttgttaaggctcccagaagacctcttaatgctgcttctaacctctgagaaaattcgtaaaatttctttaatttgcctactagtggaacaactgcaccccatgccttctcttgcaacttctcatctgctggatgctggattgcctctcgtatttcgtggccagctcctctgtatgactgcaagtcctccaagatgccttctgcatcttttaatactacattcacctgattataaatttccttctcagactctgtaggctgggcattttcaaagtccaagaaaaaatgtgctgcattgtggtctatgtccctggttagcaccttaatgagattacccatgccagcaaacctccccagagtgagagtctctggtgcctcttccagtcaccaaacagcagcaaaaaagcaaggaacttaaggacctactgccaagtaaacaggccttgtggcagtgaaaggataaactgtccatcattctttcttctcctcggagatttcacaggaaaaggagaaagcgcaggaaacaggaggccttcagccagtgctggtgattctgtccttgtccttctatccttggattggcgttccctctttcctagttcacttgttccagtccttcaacttctgtttcttgctaacaggtgtgcaaatgaattaccctccgctcgagcctccaggcgctctcagtcccgctcctgcgccctcctggagccgcagaggcggctcctcagcggcgctagggggagccccgggtccggagcgggggagcggcggcagccggaccgggagcccctcaacacctgcccctgtggcagagccgcgacaagccaggcggcagctccgagcggggagggcaagtgac

SEQ ID NO: 18504 - RNA, 3298 nt, Homo sapiens
  source 1..3298: mol_type = other RNA
tgagctgctgtaccaaaataccacaaactgcatggcttaaaacaacagaaatttattccctcacaatcctggaggccagatgtctgaaatcaagatattggtagggttggttccttctcgagactctgagggagaatctgtgacatgcctgttttcctagcttctagtgacttcctccaattcttagggttctttggctcatagatgcattgctctaatctctgcctccatcttcccatggccttcagctctgtgtgtctatttccccttcttttctaagagctagtcattgaatttagggcccaccctactacaggttgatctcatttccaggtccttgatttcatctgcaaaaactttttccaaataatgtcacacgtggagattcccagtgaatgtatctcctgggggccactattcagcctattacactattcttagaagatgcctagaaggatatggccaatgttatccagaaggcttcatgaaggaggtaatagaagctaacccttcaaagatgaaagttggcgttcattagagggtcacaaggggaggaagggaatgtcaggttcagggaccagccagaccagagctaaggaagtgacatcacatggaacaatttgtgaacagcaagcagtagggcctggctgcaggacagggtgtgaagtgggggagcagtgatcaggagggccagagagatcagcagggatgtgatcttgagaagctgtgtgtgccatgatctggccctattaatccagaagggtctgatggaagcctctgtgattctcttccatggttaaacattttaattgtattatacctcggatattcctaaatatttaaaacactggcatggttgaactagacaacctttaagtagtttgttccaaccatgagatttagatttcatgatttaggttttatgatcttaaactgaaacctgttagttttctaccactagtgagatcatggcctctgcttttctcctgggaagtccctcttataatcactctcttcccatgattaaagggctactctgccttcatgttgctacccgctcccctggaaatggagaatcaagcaaggatgcggttttccttccattactacatccatacaagagtaaatcaagaataaaagtccagttaatgaaaagatcactggtcttaatatacttagcaaaattttaaaggcaattaaaagtatatacatagacaatgatcaaaattctaatgaaaagacccggctctcccctaaaagaagaaaaaatcatgtaatgtatatatgcattccataaaaacatacatggggaaaacttcagaagcctaaaaacaaaacatcagtaaaccaagccacacttagaaaaatgaaagctgatttttattttatcatcaacagccattctttagacatgaacatgcatacgtaatattctacgcacacatcacagcttttaacgttagttaataaaggttaaacacacaacatacatccttacaaaaaaagtcaaaatgcaaacttaaaactttaaacaaaagtattactaatttaaaaaaagtttgtgttgggtaccatttgtacaacacagttaatttaaacattttcattttggttgcacatgaaaaaggcggcagtagaaaataaagtcattgagggtttttaaatagcagaataggcagttttgccatgcaggagaagcaatattaaatattagtttcaaaaaaaatccacatttaaaaatatttagttcaagtcacagaatttttctcagtagagaccccaatgcaatgcataattagctgccttagatggcccgtttgaaaggatgatatcccttcagagtgtaactttactgattttggcacagaaaagaagtcttaagaacatgattaaaaaagagggaagaggaacagaggaaagaaataaaagcaagaataaatgagatagtaattgcaatcactaaaaaactgcattctcagtcattgcagaatactgtcttctgtctacagcaggtgcttattccagaattgttattgcagcatggatttaatttgcttggaggtagtctcatcattcaaatgttttgttgtgtacctgagagcatttagaagaccttccacactattaggaggttggtccttaagaactttgatacaacctttcatatcaattttggaagttttagcaaatgctcccactggatgtacgtggtcatagagtattatgacacccaccattaccctcaagcagaatgacactgtctcttcatttgtaaatctgcttctgtattccggtgtttccagcatgactctgcatacactagccattgtgcttaaacaatctgtggtattttctattggtaaatttttattctctgatacaaattttgttgtggcatcactcaaggttttcagcattggagttgcctcagcataaaacaaagacattcgatttgccaattcattatttacttcattttctccttctgccggtacattgttaatcctcatacgactcaatgttcttctataatagctgaaatcattctgtatggcaggatttgtcatcttgagttcatcaaaccggagtgtgaaatgaagaatttctgcaaactgtttagcaagagcctgctctcgctctagatgctgggtgggagaatatggggtacttgttaaggctcccagaagacctcttaatgctgcttctaacctctgagaaaattcgtaaaatttctttaatttgcctactagtggaacaactgcaccccatgccttctcttgcaacttctcatctgctggatgctggattgcctctcgtatttcgtggccagctcctctgtatgactgcaagtcctccaagatgccttctgcatcttttaatactacattcacctgattataaatttccttctcagactctgtaggctgggcattttcaaagtccaagaaaaaatgtgctgcattgtggtctatgtccctggttagcaccttaatgagattacccatgccagcaaaccttcagccagtgctggtgattctgtccttgtccttctatcaactgggtaaccttgaatgagttaatcaaattccaggcctcagtttcttctcctggcggcccgggcgggcgaggggagcgcggcgcgggagcgcaggagcctcggagcctccggtgccgccgccgccgccgtttccgggttggcggggctcacgtcaccgccacaggtttgcgagctgcccccgccgcggcggcagcagcagcagcagcagcagcccgggcgagtgccaggcgagaaataact

SEQ ID NO: 18505 - RNA, 3198 nt, Homo sapiens
  source 1..3198: mol_type = other RNA
tgagctgctgtaccaaaataccacaaactgcatggcttaaaacaacagaaatttattccctcacaatcctggaggccagatgtctgaaatcaagatattggtagggttggttccttctcgagactctgagggagaatctgtgacatgcctgttttcctagcttctagtgacttcctccaattcttagggttctttggctcatagatgcattgctctaatctctgcctccatcttcccatggccttcagctctgtgtgtctatttccccttcttttctaagagctagtcattgaatttagggcccaccctactacaggttgatctcatttccaggtccttgatttcatctgcaaaaactttttccaaataatgtcacacgtggagattcccagtgaatgtatctcctgggggccactattcagcctattacactattcttagaagatgcctagaaggatatggccaatgttatccagaaggcttcatgaaggaggtaatagaagctaacccttcaaagatgaaagttggcgttcattagagggtcacaaggggaggaagggaatgtcaggttcagggaccagccagaccagagctaaggaagtgacatcacatggaacaatttgtgaacagcaagcagtagggcctggctgcaggacagggtgtgaagtgggggagcagtgatcaggagggccagagagatcagcagggatgtgatcttgagaagctgtgtgtgccatgatctggccctattaatccagaagggtctgatggaagcctctgtgattctcttccatggttaaacattttaattgtattatacctcggatattcctaaatatttaaaacactggcatggttgaactagacaacctttaagtagtttgttccaaccatgagatttagatttcatgatttaggttttatgatcttaaactgaaacctgttagttttctaccactagtgagatcatggcctctgcttttctcctgggaagtccctcttataatcactctcttcccatgattaaagggctactctgccttcatgttgctacccgctcccctggaaatggagaatcaagcaaggatgcggttttccttccattactacatccatacaagagtaaatcaagaataaaagtccagttaatgaaaagatcactggtcttaatatacttagcaaaattttaaaggcaattaaaagtatatacatagacaatgatcaaaattctaatgaaaagacccggctctcccctaaaagaagaaaaaatcatgtaatgtatatatgcattccataaaaacatacatggggaaaacttcagaagcctaaaaacaaaacatcagtaaaccaagccacacttagaaaaatgaaagctgatttttattttatcatcaacagccattctttagacatgaacatgcatacgtaatattctacgcacacatcacagcttttaacgttagttaataaaggttaaacacacaacatacatccttacaaaaaaagtcaaaatgcaaacttaaaactttaaacaaaagtattactaatttaaaaaaagtttgtgttgggtaccatttgtacaacacagttaatttaaacattttcattttggttgcacatgaaaaaggcggcagtagaaaataaagtcattgagggtttttaaatagcagaataggcagttttgccatgcaggagaagcaatattaaatattagtttcaaaaaaaatccacatttaaaaatatttagttcaagtcacagaatttttctcagtagagaccccaatgcaatgcataattagctgccttagatggcccgtttgaaaggatgatatcccttcagagtgtaactttactgattttggcacagaaaagaagtcttaagaacatgattaaaaaagagggaagaggaacagaggaaagaaataaaagcaagaataaatgagatagtaattgcaatcactaaaaaactgcattctcagtcattgcagaatactgtcttctgtctacagcaggtgcttattccagaattgttattgcagcatggatttaatttgcttggaggtagtctcatcattcaaatgttttgttgtgtacctgagagcatttagaagaccttccacactattaggaggttggtccttaagaactttgatacaacctttcatatcaattttggaagttttagcaaatgctcccactggatgtacgtggtcatagagtattatgacacccaccattaccctcaagcagaatgacactgtctcttcatttgtaaatctgcttctgtattccggtgtttccagcatgactctgcatacactagccattgtgcttaaacaatctgtggtattttctattggtaaatttttattctctgatacaaattttgttgtggcatcactcaaggttttcagcattggagttgcctcagcataaaacaaagacattcgatttgccaattcattatttacttcattttctccttctgccggtacattgttaatcctcatacgactcaatgttcttctataatagctgaaatcattctgtatggcaggatttgtcatcttgagttcatcaaaccggagtgtgaaatgaagaatttctgcaaactgtttagcaagagcctgctctcgctctagatgctgggtgggagaatatggggtacttgttaaggctcccagaagacctcttaatgctgcttctaacctctgagaaaattcgtaaaatttctttaatttgcctactagtggaacaactgcaccccatgccttctcttgcaacttctcatctgctggatgctggattgcctctcgtatttcgtggccagctcctctgtatgactgcaagtcctccaagatgccttctgcatcttttaatactacattcacctgattataaatttccttctcagactctgtaggctgggcattttcaaagtccaagaaaaaatgtgctgcattgtggtctatgtccctggttagcaccttaatgagattacccatgccagcaaaccttcagccagtgctggtgattctgtccttgtccttctatcaactgggtaaccttgaatgagttaatcaaattccaggcctcagtttcttctccttcgagaagccgagccgccggcgctcgcacaaaaggaggacgctcgcctcgcgacgcgcctccccccgcgcccagtccccgccgcatcgc

SEQ ID NO: 18506 - RNA, 3258 nt, Homo sapiens
  source 1..3258: mol_type = other RNA
tgagctgctgtaccaaaataccacaaactgcatggcttaaaacaacagaaatttattccctcacaatcctggaggccagatgtctgaaatcaagatattggtagggttggttccttctcgagactctgagggagaatctgtgacatgcctgttttcctagcttctagtgacttcctccaattcttagggttctttggctcatagatgcattgctctaatctctgcctccatcttcccatggccttcagctctgtgtgtctatttccccttcttttctaagagctagtcattgaatttagggcccaccctactacaggttgatctcatttccaggtccttgatttcatctgcaaaaactttttccaaataatgtcacacgtggagattcccagtgaatgtatctcctgggggccactattcagcctattacactattcttagaagatgcctagaaggatatggccaatgttatccagaaggcttcatgaaggaggtaatagaagctaacccttcaaagatgaaagttggcgttcattagagggtcacaaggggaggaagggaatgtcaggttcagggaccagccagaccagagctaaggaagtgacatcacatggaacaatttgtgaacagcaagcagtagggcctggctgcaggacagggtgtgaagtgggggagcagtgatcaggagggccagagagatcagcagggatgtgatcttgagaagctgtgtgtgccatgatctggccctattaatccagaagggtctgatggaagcctctgtgattctcttccatggttaaacattttaattgtattatacctcggatattcctaaatatttaaaacactggcatggttgaactagacaacctttaagtagtttgttccaaccatgagatttagatttcatgatttaggttttatgatcttaaactgaaacctgttagttttctaccactagtgagatcatggcctctgcttttctcctgggaagtccctcttataatcactctcttcccatgattaaagggctactctgccttcatgttgctacccgctcccctggaaatggagaatcaagcaaggatgcggttttccttccattactacatccatacaagagtaaatcaagaataaaagtccagttaatgaaaagatcactggtcttaatatacttagcaaaattttaaaggcaattaaaagtatatacatagacaatgatcaaaattctaatgaaaagacccggctctcccctaaaagaagaaaaaatcatgtaatgtatatatgcattccataaaaacatacatggggaaaacttcagaagcctaaaaacaaaacatcagtaaaccaagccacacttagaaaaatgaaagctgatttttattttatcatcaacagccattctttagacatgaacatgcatacgtaatattctacgcacacatcacagcttttaacgttagttaataaaggttaaacacacaacatacatccttacaaaaaaagtcaaaatgcaaacttaaaactttaaacaaaagtattactaatttaaaaaaagtttgtgttgggtaccatttgtacaacacagttaatttaaacattttcattttggttgcacatgaaaaaggcggcagtagaaaataaagtcattgagggtttttaaatagcagaataggcagttttgccatgcaggagaagcaatattaaatattagtttcaaaaaaaatccacatttaaaaatatttagttcaagtcacagaatttttctcagtagagaccccaatgcaatgcataattagctgccttagatggcccgtttgaaaggatgatatcccttcagagtgtaactttactgattttggcacagaaaagaagtcttaagaacatgattaaaaaagagggaagaggaacagaggaaagaaataaaagcaagaataaatgagatagtaattgcaatcactaaaaaactgcattctcagtcattgcagaatactgtcttctgtctacagcaggtgcttattccagaattgttattgcagcatggatttaatttgcttggaggtagtctcatcattcaaatgttttgttgtgtacctgagagcatttagaagaccttccacactattaggaggttggtccttaagaactttgatacaacctttcatatcaattttggaagttttagcaaatgctcccactggatgtacgtggtcatagagtattatgacacccaccattaccctcaagcagaatgacactgtctcttcatttgtaaatctgcttctgtattccggtgtttccagcatgactctgcatacactagccattgtgcttaaacaatctgtggtattttctattggtaaatttttattctctgatacaaattttgttgtggcatcactcaaggttttcagcattggagttgcctcagcataaaacaaagacattcgatttgccaattcattatttacttcattttctccttctgccggtacattgttaatcctcatacgactcaatgttcttctataatagctgaaatcattctgtatggcaggatttgtcatcttgagttcatcaaaccggagtgtgaaatgaagaatttctgcaaactgtttagcaagagcctgctctcgctctagatgctgggtgggagaatatggggtacttgttaaggctcccagaagacctcttaatgctgcttctaacctctgagaaaattcgtaaaatttctttaatttgcctactagtggaacaactgcaccccatgccttctcttgcaacttctcatctgctggatgctggattgcctctcgtatttcgtggccagctcctctgtatgactgcaagtcctccaagatgccttctgcatcttttaatactacattcacctgattataaatttccttctcagactctgtaggctgggcattttcaaagtccaagaaaaaatgtgctgcattgtggtctatgtccctggttagcaccttaatgagattacccatgccagcaaaccttcagccagtgctggtgattctgtccttgtccttctatcctccgctcgagcctccaggcgctctcagtcccgctcctgcgccctcctggagccgcagaggcggctcctcagcggcgctagggggagccccgggtccggagcgggggagcggcggcagccggaccgggagcccctcaacacctgcccctgtggcagagccgcgacaagccaggcggcagctccgagcggggagggcaagtgac

SEQ ID NO: 18507 - RNA, 3385 nt, Homo sapiens
  source 1..3385: mol_type = other RNA
tgagctgctgtaccaaaataccacaaactgcatggcttaaaacaacagaaatttattccctcacaatcctggaggccagatgtctgaaatcaagatattggtagggttggttccttctcgagactctgagggagaatctgtgacatgcctgttttcctagcttctagtgacttcctccaattcttagggttctttggctcatagatgcattgctctaatctctgcctccatcttcccatggccttcagctctgtgtgtctatttccccttcttttctaagagctagtcattgaatttagggcccaccctactacaggttgatctcatttccaggtccttgatttcatctgcaaaaactttttccaaataatgtcacacgtggagattcccagtgaatgtatctcctgggggccactattcagcctattacactattcttagaagatgcctagaaggatatggccaatgttatccagaaggcttcatgaaggaggtaatagaagctaacccttcaaagatgaaagttggcgttcattagagggtcacaaggggaggaagggaatgtcaggttcagggaccagccagaccagagctaaggaagtgacatcacatggaacaatttgtgaacagcaagcagtagggcctggctgcaggacagggtgtgaagtgggggagcagtgatcaggagggccagagagatcagcagggatgtgatcttgagaagctgtgtgtgccatgatctggccctattaatccagaagggtctgatggaagcctctgtgattctcttccatggttaaacattttaattgtattatacctcggatattcctaaatatttaaaacactggcatggttgaactagacaacctttaagtagtttgttccaaccatgagatttagatttcatgatttaggttttatgatcttaaactgaaacctgttagttttctaccactagtgagatcatggcctctgcttttctcctgggaagtccctcttataatcactctcttcccatgattaaagggctactctgccttcatgttgctacccgctcccctggaaatggagaatcaagcaaggatgcggttttccttccattactacatccatacaagagtaaatcaagaataaaagtccagttaatgaaaagatcactggtcttaatatacttagcaaaattttaaaggcaattaaaagtatatacatagacaatgatcaaaattctaatgaaaagacccggctctcccctaaaagaagaaaaaatcatgtaatgtatatatgcattccataaaaacatacatggggaaaacttcagaagcctaaaaacaaaacatcagtaaaccaagccacacttagaaaaatgaaagctgatttttattttatcatcaacagccattctttagacatgaacatgcatacgtaatattctacgcacacatcacagcttttaacgttagttaataaaggttaaacacacaacatacatccttacaaaaaaagtcaaaatgcaaacttaaaactttaaacaaaagtattactaatttaaaaaaagtttgtgttgggtaccatttgtacaacacagttaatttaaacattttcattttggttgcacatgaaaaaggcggcagtagaaaataaagtcattgagggtttttaaatagcagaataggcagttttgccatgcaggagaagcaatattaaatattagtttcaaaaaaaatccacatttaaaaatatttagttcaagtcacagaatttttctcagtagagaccccaatgcaatgcataattagctgccttagatggcccgtttgaaaggatgatatcccttcagagtgtaactttactgattttggcacagaaaagaagtcttaagaacatgattaaaaaagagggaagaggaacagaggaaagaaataaaagcaagaataaatgagatagtaattgcaatcactaaaaaactgcattctcagtcattgcagaatactgtcttctgtctacagcaggtgcttattccagaattgttattgcagcatggatttaatttgcttggaggtagtctcatcattcaaatgttttgttgtgtacctgagagcatttagaagaccttccacactattaggaggttggtccttaagaactttgatacaacctttcatatcaattttggaagttttagcaaatgctcccactggatgtacgtggtcatagagtattatgacacccaccattaccctcaagcagaatgacactgtctcttcatttgtaaatctgcttctgtattccggtgtttccagcatgactctgcatacactagccattgtgcttaaacaatctgtggtattttctattggtaaatttttattctctgatacaaattttgttgtggcatcactcaaggttttcagcattggagttgcctcagcataaaacaaagacattcgatttgccaattcattatttacttcattttctccttctgccggtacattgttaatcctcatacgactcaatgttcttctataatagctgaaatcattctgtatggcaggatttgtcatcttgagttcatcaaaccggagtgtgaaatgaagaatttctgcaaactgtttagcaagagcctgctctcgctctagatgctgggtgggagaatatggggtacttgttaaggctcccagaagacctcttaatgctgcttctaacctctgagaaaattcgtaaaatttctttaatttgcctactagtggaacaactgcaccccatgccttctcttgcaacttctcatctgctggatgctggattgcctctcgtatttcgtggccagctcctctgtatgactgcaagtcctccaagatgccttctgcatcttttaatactacattcacctgattataaatttccttctcagactctgtaggctgggcattttcaaagtccaagaaaaaatgtgctgcattgtggtctatgtccctggttagcaccttaatgagattacccatgccagcaaaccttcagccagtgctggtgattctgtccttgtccttctatccttggattggcgttccctctttcctagttcacttgttccagtccttcaacttctgtttcttgctaacaggtgtgcaaatgaattaccaactgggtaaccttgaatgagttaatcaaattccaggcctcagtttcttctcctggcggcccgggcgggcgaggggagcgcggcgcgggagcgcaggagcctcggagcctccggtgccgccgccgccgccgtttccgggttggcggggctcacgtcaccgccacaggtttgcgagctgcccccgccgcggcggcagcagcagcagcagcagcagcccgggcgagtgccaggcgagaaataact

SEQ ID NO: 18508 - RNA, 3285 nt, Homo sapiens
  source 1..3285: mol_type = other RNA
tgagctgctgtaccaaaataccacaaactgcatggcttaaaacaacagaaatttattccctcacaatcctggaggccagatgtctgaaatcaagatattggtagggttggttccttctcgagactctgagggagaatctgtgacatgcctgttttcctagcttctagtgacttcctccaattcttagggttctttggctcatagatgcattgctctaatctctgcctccatcttcccatggccttcagctctgtgtgtctatttccccttcttttctaagagctagtcattgaatttagggcccaccctactacaggttgatctcatttccaggtccttgatttcatctgcaaaaactttttccaaataatgtcacacgtggagattcccagtgaatgtatctcctgggggccactattcagcctattacactattcttagaagatgcctagaaggatatggccaatgttatccagaaggcttcatgaaggaggtaatagaagctaacccttcaaagatgaaagttggcgttcattagagggtcacaaggggaggaagggaatgtcaggttcagggaccagccagaccagagctaaggaagtgacatcacatggaacaatttgtgaacagcaagcagtagggcctggctgcaggacagggtgtgaagtgggggagcagtgatcaggagggccagagagatcagcagggatgtgatcttgagaagctgtgtgtgccatgatctggccctattaatccagaagggtctgatggaagcctctgtgattctcttccatggttaaacattttaattgtattatacctcggatattcctaaatatttaaaacactggcatggttgaactagacaacctttaagtagtttgttccaaccatgagatttagatttcatgatttaggttttatgatcttaaactgaaacctgttagttttctaccactagtgagatcatggcctctgcttttctcctgggaagtccctcttataatcactctcttcccatgattaaagggctactctgccttcatgttgctacccgctcccctggaaatggagaatcaagcaaggatgcggttttccttccattactacatccatacaagagtaaatcaagaataaaagtccagttaatgaaaagatcactggtcttaatatacttagcaaaattttaaaggcaattaaaagtatatacatagacaatgatcaaaattctaatgaaaagacccggctctcccctaaaagaagaaaaaatcatgtaatgtatatatgcattccataaaaacatacatggggaaaacttcagaagcctaaaaacaaaacatcagtaaaccaagccacacttagaaaaatgaaagctgatttttattttatcatcaacagccattctttagacatgaacatgcatacgtaatattctacgcacacatcacagcttttaacgttagttaataaaggttaaacacacaacatacatccttacaaaaaaagtcaaaatgcaaacttaaaactttaaacaaaagtattactaatttaaaaaaagtttgtgttgggtaccatttgtacaacacagttaatttaaacattttcattttggttgcacatgaaaaaggcggcagtagaaaataaagtcattgagggtttttaaatagcagaataggcagttttgccatgcaggagaagcaatattaaatattagtttcaaaaaaaatccacatttaaaaatatttagttcaagtcacagaatttttctcagtagagaccccaatgcaatgcataattagctgccttagatggcccgtttgaaaggatgatatcccttcagagtgtaactttactgattttggcacagaaaagaagtcttaagaacatgattaaaaaagagggaagaggaacagaggaaagaaataaaagcaagaataaatgagatagtaattgcaatcactaaaaaactgcattctcagtcattgcagaatactgtcttctgtctacagcaggtgcttattccagaattgttattgcagcatggatttaatttgcttggaggtagtctcatcattcaaatgttttgttgtgtacctgagagcatttagaagaccttccacactattaggaggttggtccttaagaactttgatacaacctttcatatcaattttggaagttttagcaaatgctcccactggatgtacgtggtcatagagtattatgacacccaccattaccctcaagcagaatgacactgtctcttcatttgtaaatctgcttctgtattccggtgtttccagcatgactctgcatacactagccattgtgcttaaacaatctgtggtattttctattggtaaatttttattctctgatacaaattttgttgtggcatcactcaaggttttcagcattggagttgcctcagcataaaacaaagacattcgatttgccaattcattatttacttcattttctccttctgccggtacattgttaatcctcatacgactcaatgttcttctataatagctgaaatcattctgtatggcaggatttgtcatcttgagttcatcaaaccggagtgtgaaatgaagaatttctgcaaactgtttagcaagagcctgctctcgctctagatgctgggtgggagaatatggggtacttgttaaggctcccagaagacctcttaatgctgcttctaacctctgagaaaattcgtaaaatttctttaatttgcctactagtggaacaactgcaccccatgccttctcttgcaacttctcatctgctggatgctggattgcctctcgtatttcgtggccagctcctctgtatgactgcaagtcctccaagatgccttctgcatcttttaatactacattcacctgattataaatttccttctcagactctgtaggctgggcattttcaaagtccaagaaaaaatgtgctgcattgtggtctatgtccctggttagcaccttaatgagattacccatgccagcaaaccttcagccagtgctggtgattctgtccttgtccttctatccttggattggcgttccctctttcctagttcacttgttccagtccttcaacttctgtttcttgctaacaggtgtgcaaatgaattaccaactgggtaaccttgaatgagttaatcaaattccaggcctcagtttcttctccttcgagaagccgagccgccggcgctcgcacaaaaggaggacgctcgcctcgcgacgcgcctccccccgcgcccagtccccgccgcatcgc

SEQ ID NO: 18509 - RNA, 3345 nt, Homo sapiens
  source 1..3345: mol_type = other RNA
tgagctgctgtaccaaaataccacaaactgcatggcttaaaacaacagaaatttattccctcacaatcctggaggccagatgtctgaaatcaagatattggtagggttggttccttctcgagactctgagggagaatctgtgacatgcctgttttcctagcttctagtgacttcctccaattcttagggttctttggctcatagatgcattgctctaatctctgcctccatcttcccatggccttcagctctgtgtgtctatttccccttcttttctaagagctagtcattgaatttagggcccaccctactacaggttgatctcatttccaggtccttgatttcatctgcaaaaactttttccaaataatgtcacacgtggagattcccagtgaatgtatctcctgggggccactattcagcctattacactattcttagaagatgcctagaaggatatggccaatgttatccagaaggcttcatgaaggaggtaatagaagctaacccttcaaagatgaaagttggcgttcattagagggtcacaaggggaggaagggaatgtcaggttcagggaccagccagaccagagctaaggaagtgacatcacatggaacaatttgtgaacagcaagcagtagggcctggctgcaggacagggtgtgaagtgggggagcagtgatcaggagggccagagagatcagcagggatgtgatcttgagaagctgtgtgtgccatgatctggccctattaatccagaagggtctgatggaagcctctgtgattctcttccatggttaaacattttaattgtattatacctcggatattcctaaatatttaaaacactggcatggttgaactagacaacctttaagtagtttgttccaaccatgagatttagatttcatgatttaggttttatgatcttaaactgaaacctgttagttttctaccactagtgagatcatggcctctgcttttctcctgggaagtccctcttataatcactctcttcccatgattaaagggctactctgccttcatgttgctacccgctcccctggaaatggagaatcaagcaaggatgcggttttccttccattactacatccatacaagagtaaatcaagaataaaagtccagttaatgaaaagatcactggtcttaatatacttagcaaaattttaaaggcaattaaaagtatatacatagacaatgatcaaaattctaatgaaaagacccggctctcccctaaaagaagaaaaaatcatgtaatgtatatatgcattccataaaaacatacatggggaaaacttcagaagcctaaaaacaaaacatcagtaaaccaagccacacttagaaaaatgaaagctgatttttattttatcatcaacagccattctttagacatgaacatgcatacgtaatattctacgcacacatcacagcttttaacgttagttaataaaggttaaacacacaacatacatccttacaaaaaaagtcaaaatgcaaacttaaaactttaaacaaaagtattactaatttaaaaaaagtttgtgttgggtaccatttgtacaacacagttaatttaaacattttcattttggttgcacatgaaaaaggcggcagtagaaaataaagtcattgagggtttttaaatagcagaataggcagttttgccatgcaggagaagcaatattaaatattagtttcaaaaaaaatccacatttaaaaatatttagttcaagtcacagaatttttctcagtagagaccccaatgcaatgcataattagctgccttagatggcccgtttgaaaggatgatatcccttcagagtgtaactttactgattttggcacagaaaagaagtcttaagaacatgattaaaaaagagggaagaggaacagaggaaagaaataaaagcaagaataaatgagatagtaattgcaatcactaaaaaactgcattctcagtcattgcagaatactgtcttctgtctacagcaggtgcttattccagaattgttattgcagcatggatttaatttgcttggaggtagtctcatcattcaaatgttttgttgtgtacctgagagcatttagaagaccttccacactattaggaggttggtccttaagaactttgatacaacctttcatatcaattttggaagttttagcaaatgctcccactggatgtacgtggtcatagagtattatgacacccaccattaccctcaagcagaatgacactgtctcttcatttgtaaatctgcttctgtattccggtgtttccagcatgactctgcatacactagccattgtgcttaaacaatctgtggtattttctattggtaaatttttattctctgatacaaattttgttgtggcatcactcaaggttttcagcattggagttgcctcagcataaaacaaagacattcgatttgccaattcattatttacttcattttctccttctgccggtacattgttaatcctcatacgactcaatgttcttctataatagctgaaatcattctgtatggcaggatttgtcatcttgagttcatcaaaccggagtgtgaaatgaagaatttctgcaaactgtttagcaagagcctgctctcgctctagatgctgggtgggagaatatggggtacttgttaaggctcccagaagacctcttaatgctgcttctaacctctgagaaaattcgtaaaatttctttaatttgcctactagtggaacaactgcaccccatgccttctcttgcaacttctcatctgctggatgctggattgcctctcgtatttcgtggccagctcctctgtatgactgcaagtcctccaagatgccttctgcatcttttaatactacattcacctgattataaatttccttctcagactctgtaggctgggcattttcaaagtccaagaaaaaatgtgctgcattgtggtctatgtccctggttagcaccttaatgagattacccatgccagcaaaccttcagccagtgctggtgattctgtccttgtccttctatccttggattggcgttccctctttcctagttcacttgttccagtccttcaacttctgtttcttgctaacaggtgtgcaaatgaattaccctccgctcgagcctccaggcgctctcagtcccgctcctgcgccctcctggagccgcagaggcggctcctcagcggcgctagggggagccccgggtccggagcgggggagcggcggcagccggaccgggagcccctcaacacctgcccctgtggcagagccgcgacaagccaggcggcagctccgagcggggagggcaagtgac

SEQ ID NO: 18510 - RNA, 3431 nt, Homo sapiens
  source 1..3431: mol_type = other RNA
tgagctgctgtaccaaaataccacaaactgcatggcttaaaacaacagaaatttattccctcacaatcctggaggccagatgtctgaaatcaagatattggtagggttggttccttctcgagactctgagggagaatctgtgacatgcctgttttcctagcttctagtgacttcctccaattcttagggttctttggctcatagatgcattgctctaatctctgcctccatcttcccatggccttcagctctgtgtgtctatttccccttcttttctaagagctagtcattgaatttagggcccaccctactacaggttgatctcatttccaggtccttgatttcatctgcaaaaactttttccaaataatgtcacacgtggagattcccagtgaatgtatctcctgggggccactattcagcctattacactattcttagaagatgcctagaaggatatggccaatgttatccagaaggcttcatgaaggaggtaatagaagctaacccttcaaagatgaaagttggcgttcattagagggtcacaaggggaggaagggaatgtcaggttcagggaccagccagaccagagctaaggaagtgacatcacatggaacaatttgtgaacagcaagcagtagggcctggctgcaggacagggtgtgaagtgggggagcagtgatcaggagggccagagagatcagcagggatgtgatcttgagaagctgtgtgtgccatgatctggccctattaatccagaagggtctgatggaagcctctgtgattctcttccatggttaaacattttaattgtattatacctcggatattcctaaatatttaaaacactggcatggttgaactagacaacctttaagtagtttgttccaaccatgagatttagatttcatgatttaggttttatgatcttaaactgaaacctgttagttttctaccactagtgagatcatggcctctgcttttctcctgggaagtccctcttataatcactctcttcccatgattaaagggctactctgccttcatgttgctacccgctcccctggaaatggagaatcaagcaaggatgcggttttccttccattactacatccatacaagagtaaatcaagaataaaagtccagttaatgaaaagatcactggtcttaatatacttagcaaaattttaaaggcaattaaaagtatatacatagacaatgatcaaaattctaatgaaaagacccggctctcccctaaaagaagaaaaaatcatgtaatgtatatatgcattccataaaaacatacatggggaaaacttcagaagcctaaaaacaaaacatcagtaaaccaagccacacttagaaaaatgaaagctgatttttattttatcatcaacagccattctttagacatgaacatgcatacgtaatattctacgcacacatcacagcttttaacgttagttaataaaggttaaacacacaacatacatccttacaaaaaaagtcaaaatgcaaacttaaaactttaaacaaaagtattactaatttaaaaaaagtttgtgttgggtaccatttgtacaacacagttaatttaaacattttcattttggttgcacatgaaaaaggcggcagtagaaaataaagtcattgagggtttttaaatagcagaataggcagttttgccatgcaggagaagcaatattaaatattagtttcaaaaaaaatccacatttaaaaatatttagttcaagtcacagaatttttctcagtagagaccccaatgcaatgcataattagctgccttagatggcccgtttgaaaggatgatatcccttcagagtgtaactttactgattttggcacagaaaagaagtcttaagaacatgattaaaaaagagggaagaggaacagaggaaagaaataaaagcaagaataaatgagatagtaattgcaatcactaaaaaactgcattctcagtcattgcagaatactgtcttctgtctacagcaggtgcttattccagaattgttattgcagcatggatttaatttgcttggaggtagtctcatcattcaaatgttttgttgtgtacctgagagcatttagaagaccttccacactattaggaggttggtccttaagaactttgatacaacctttcatatcaattttggaagttttagcaaatgctcccactggatgtacgtggtcatagagtattatgacacccaccattaccctcaagcagaatgacactgtctcttcatttgtaaatctgcttctgtattccggtgtttccagcatgactctgcatacactagccattgtgcttaaacaatctgtggtattttctattggtaaatttttattctctgatacaaattttgttgtggcatcactcaaggttttcagcattggagttgcctcagcataaaacaaagacattcgatttgccaattcattatttacttcattttctccttctgccggtacattgttaatcctcatacgactcaatgttcttctataatagctgaaatcattctgtatggcaggatttgtcatcttgagttcatcaaaccggagtgtgaaatgaagaatttctgcaaactgtttagcaagagcctgctctcgctctagatgctgggtgggagaatatggggtacttgttaaggctcccagaagacctcttaatgctgcttctaacctctgagaaaattcgtaaaatttctttaatttgcctactagtggaacaactgcaccccatgccttctcttgcaacttctcatctgctggatgctggattgcctctcgtatttcgtggccagctcctctgtatgactgcaagtcctccaagatgccttctgcatcttttaatactacattcacctgattataaatttccttctcagactctgtaggctgggcattttcaaagtccaagaaaaaatgtgctgcattgtggtctatgtccctggttagcaccttaatgagattacccatgccagcaaaccttcagccagtgctggtgattctgtccttgtccttctatccttggattggcgttccctctttcctagttcacttgttccagtccttcaacttctgtttcttgctaacaggtgtgcaaatgaattacctgagaagtgcaaggttggttcagaatacctactgttttcaccacccaactgggtaaccttgaatgagttaatcaaattccaggcctcagtttcttctcctggcggcccgggcgggcgaggggagcgcggcgcgggagcgcaggagcctcggagcctccggtgccgccgccgccgccgtttccgggttggcggggctcacgtcaccgccacaggtttgcgagctgcccccgccgcggcggcagcagcagcagcagcagcagcccgggcgagtgccaggcgagaaataact

SEQ ID NO: 18511 - RNA, 3390 nt, Homo sapiens
  source 1..3390: mol_type = other RNA
tgagctgctgtaccaaaataccacaaactgcatggcttaaaacaacagaaatttattccctcacaatcctggaggccagatgtctgaaatcaagatattggtagggttggttccttctcgagactctgagggagaatctgtgacatgcctgttttcctagcttctagtgacttcctccaattcttagggttctttggctcatagatgcattgctctaatctctgcctccatcttcccatggccttcagctctgtgtgtctatttccccttcttttctaagagctagtcattgaatttagggcccaccctactacaggttgatctcatttccaggtccttgatttcatctgcaaaaactttttccaaataatgtcacacgtggagattcccagtgaatgtatctcctgggggccactattcagcctattacactattcttagaagatgcctagaaggatatggccaatgttatccagaaggcttcatgaaggaggtaatagaagctaacccttcaaagatgaaagttggcgttcattagagggtcacaaggggaggaagggaatgtcaggttcagggaccagccagaccagagctaaggaagtgacatcacatggaacaatttgtgaacagcaagcagtagggcctggctgcaggacagggtgtgaagtgggggagcagtgatcaggagggccagagagatcagcagggatgtgatcttgagaagctgtgtgtgccatgatctggccctattaatccagaagggtctgatggaagcctctgtgattctcttccatggttaaacattttaattgtattatacctcggatattcctaaatatttaaaacactggcatggttgaactagacaacctttaagtagtttgttccaaccatgagatttagatttcatgatttaggttttatgatcttaaactgaaacctgttagttttctaccactagtgagatcatggcctctgcttttctcctgggaagtccctcttataatcactctcttcccatgattaaagggctactctgccttcatgttgctacccgctcccctggaaatggagaatcaagcaaggatgcggttttccttccattactacatccatacaagagtaaatcaagaataaaagtccagttaatgaaaagatcactggtcttaatatacttagcaaaattttaaaggcaattaaaagtatatacatagacaatgatcaaaattctaatgaaaagacccggctctcccctaaaagaagaaaaaatcatgtaatgtatatatgcattccataaaaacatacatggggaaaacttcagaagcctaaaaacaaaacatcagtaaaccaagccacacttagaaaaatgaaagctgatttttattttatcatcaacagccattctttagacatgaacatgcatacgtaatattctacgcacacatcacagcttttaacgttagttaataaaggttaaacacacaacatacatccttacaaaaaaagtcaaaatgcaaacttaaaactttaaacaaaagtattactaatttaaaaaaagtttgtgttgggtaccatttgtacaacacagttaatttaaacattttcattttggttgcacatgaaaaaggcggcagtagaaaataaagtcattgagggtttttaaatagcagaataggcagttttgccatgcaggagaagcaatattaaatattagtttcaaaaaaaatccacatttaaaaatatttagttcaagtcacagaatttttctcagtagagaccccaatgcaatgcataattagctgccttagatggcccgtttgaaaggatgatatcccttcagagtgtaactttactgattttggcacagaaaagaagtcttaagaacatgattaaaaaagagggaagaggaacagaggaaagaaataaaagcaagaataaatgagatagtaattgcaatcactaaaaaactgcattctcagtcattgcagaatactgtcttctgtctacagcaggtgcttattccagaattgttattgcagcatggatttaatttgcttggaggtagtctcatcattcaaatgttttgttgtgtacctgagagcatttagaagaccttccacactattaggaggttggtccttaagaactttgatacaacctttcatatcaattttggaagttttagcaaatgctcccactggatgtacgtggtcatagagtattatgacacccaccattaccctcaagcagaatgacactgtctcttcatttgtaaatctgcttctgtattccggtgtttccagcatgactctgcatacactagccattgtgcttaaacaatctgtggtattttctattggtaaatttttattctctgatacaaattttgttgtggcatcactcaaggttttcagcattggagttgcctcagcataaaacaaagacattcgatttgccaattcattatttacttcattttctccttctgccggtacattgttaatcctcatacgactcaatgttcttctataatagctgaaatcattctgtatggcaggatttgtcatcttgagttcatcaaaccggagtgtgaaatgaagaatttctgcaaactgtttagcaagagcctgctctcgctctagatgctgggtgggagaatatggggtacttgttaaggctcccagaagacctcttaatgctgcttctaacctctgagaaaattcgtaaaatttctttaatttgcctactagtggaacaactgcaccccatgccttctcttgcaacttctcatctgctggatgctggattgcctctcgtatttcgtggccagctcctctgtatgactgcaagtcctccaagatgccttctgcatcttttaatactacattcacctgattataaatttccttctcagactctgtaggctgggcattttcaaagtccaagaaaaaatgtgctgcattgtggtctatgtccctggttagcaccttaatgagattacccatgccagcaaaccttcagccagtgctggtgattctgtccttgtccttctatccttggattggcgttccctctttcctagttcacttgttccagtccttcaacttctgtttcttgctaacaggtgtgcaaatgaattacctgcttcaccactcccccagtaccactctctccacctctagtccaatgctgcagttatctggcggcccgggcgggcgaggggagcgcggcgcgggagcgcaggagcctcggagcctccggtgccgccgccgccgccgtttccgggttggcggggctcacgtcaccgccacaggtttgcgagctgcccccgccgcggcggcagcagcagcagcagcagcagcccgggcgagtgccaggcgagaaataact

SEQ ID NO: 18512 - RNA, 3332 nt, Homo sapiens
  source 1..3332: mol_type = other RNA
tgagctgctgtaccaaaataccacaaactgcatggcttaaaacaacagaaatttattccctcacaatcctggaggccagatgtctgaaatcaagatattggtagggttggttccttctcgagactctgagggagaatctgtgacatgcctgttttcctagcttctagtgacttcctccaattcttagggttctttggctcatagatgcattgctctaatctctgcctccatcttcccatggccttcagctctgtgtgtctatttccccttcttttctaagagctagtcattgaatttagggcccaccctactacaggttgatctcatttccaggtccttgatttcatctgcaaaaactttttccaaataatgtcacacgtggagattcccagtgaatgtatctcctgggggccactattcagcctattacactattcttagaagatgcctagaaggatatggccaatgttatccagaaggcttcatgaaggaggtaatagaagctaacccttcaaagatgaaagttggcgttcattagagggtcacaaggggaggaagggaatgtcaggttcagggaccagccagaccagagctaaggaagtgacatcacatggaacaatttgtgaacagcaagcagtagggcctggctgcaggacagggtgtgaagtgggggagcagtgatcaggagggccagagagatcagcagggatgtgatcttgagaagctgtgtgtgccatgatctggccctattaatccagaagggtctgatggaagcctctgtgattctcttccatggttaaacattttaattgtattatacctcggatattcctaaatatttaaaacactggcatggttgaactagacaacctttaagtagtttgttccaaccatgagatttagatttcatgatttaggttttatgatcttaaactgaaacctgttagttttctaccactagtgagatcatggcctctgcttttctcctgggaagtccctcttataatcactctcttcccatgattaaagggctactctgccttcatgttgctacccgctcccctggaaatggagaatcaagcaaggatgcggttttccttccattactacatccatacaagagtaaatcaagaataaaagtccagttaatgaaaagatcactggtcttaatatacttagcaaaattttaaaggcaattaaaagtatatacatagacaatgatcaaaattctaatgaaaagacccggctctcccctaaaagaagaaaaaatcatgtaatgtatatatgcattccataaaaacatacatggggaaaacttcagaagcctaaaaacaaaacatcagtaaaccaagccacacttagaaaaatgaaagctgatttttattttatcatcaacagccattctttagacatgaacatgcatacgtaatattctacgcacacatcacagcttttaacgttagttaataaaggttaaacacacaacatacatccttacaaaaaaagtcaaaatgcaaacttaaaactttaaacaaaagtattactaatttaaaaaaagtttgtgttgggtaccatttgtacaacacagttaatttaaacattttcattttggttgcacatgaaaaaggcggcagtagaaaataaagtcattgagggtttttaaatagcagaataggcagttttgccatgcaggagaagcaatattaaatattagtttcaaaaaaaatccacatttaaaaatatttagttcaagtcacagaatttttctcagtagagaccccaatgcaatgcataattagctgccttagatggcccgtttgaaaggatgatatcccttcagagtgtaactttactgattttggcacagaaaagaagtcttaagaacatgattaaaaaagagggaagaggaacagaggaaagaaataaaagcaagaataaatgagatagtaattgcaatcactaaaaaactgcattctcagtcattgcagaatactgtcttctgtctacagcaggtgcttattccagaattgttattgcagcatggatttaatttgcttggaggtagtctcatcattcaaatgttttgttgtgtacctgagagcatttagaagaccttccacactattaggaggttggtccttaagaactttgatacaacctttcatatcaattttggaagttttagcaaatgctcccactggatgtacgtggtcatagagtattatgacacccaccattaccctcaagcagaatgacactgtctcttcatttgtaaatctgcttctgtattccggtgtttccagcatgactctgcatacactagccattgtgcttaaacaatctgtggtattttctattggtaaatttttattctctgatacaaattttgttgtggcatcactcaaggttttcagcattggagttgcctcagcataaaacaaagacattcgatttgccaattcattatttacttcattttctccttctgccggtacattgttaatcctcatacgactcaatgttcttctataatagctgaaatcattctgtatggcaggatttgtcatcttgagttcatcaaaccggagtgtgaaatgaagaatttctgcaaactgtttagcaagagcctgctctcgctctagatgctgggtgggagaatatggggtacttgttaaggctcccagaagacctcttaatgctgcttctaacctctgagaaaattcgtaaaatttctttaatttgcctactagtggaacaactgcaccccatgccttctcttgcaacttctcatctgctggatgctggattgcctctcgtatttcgtggccagctcctctgtatgactgcaagtcctccaagatgccttctgcatcttttaatactacattcacctgattataaatttccttctcagactctgtaggctgggcattttcaaagtccaagaaaaaatgtgctgcattgtggtctatgtccctggttagcaccttaatgagattacccatgccagcaaaccttcagccagtgctggtgattctgtccttgtccttctatccttggattggcgttccctctttcctagttcacttgttccagtccttcaacttctgtttcttgctaacaggtgtgcaaatgaattacctggcggcccgggcgggcgaggggagcgcggcgcgggagcgcaggagcctcggagcctccggtgccgccgccgccgccgtttccgggttggcggggctcacgtcaccgccacaggtttgcgagctgcccccgccgcggcggcagcagcagcagcagcagcagcccgggcgagtgccaggcgagaaataact

SEQ ID NO: 18513 - RNA, 3232 nt, Homo sapiens
  source 1..3232: mol_type = other RNA
tgagctgctgtaccaaaataccacaaactgcatggcttaaaacaacagaaatttattccctcacaatcctggaggccagatgtctgaaatcaagatattggtagggttggttccttctcgagactctgagggagaatctgtgacatgcctgttttcctagcttctagtgacttcctccaattcttagggttctttggctcatagatgcattgctctaatctctgcctccatcttcccatggccttcagctctgtgtgtctatttccccttcttttctaagagctagtcattgaatttagggcccaccctactacaggttgatctcatttccaggtccttgatttcatctgcaaaaactttttccaaataatgtcacacgtggagattcccagtgaatgtatctcctgggggccactattcagcctattacactattcttagaagatgcctagaaggatatggccaatgttatccagaaggcttcatgaaggaggtaatagaagctaacccttcaaagatgaaagttggcgttcattagagggtcacaaggggaggaagggaatgtcaggttcagggaccagccagaccagagctaaggaagtgacatcacatggaacaatttgtgaacagcaagcagtagggcctggctgcaggacagggtgtgaagtgggggagcagtgatcaggagggccagagagatcagcagggatgtgatcttgagaagctgtgtgtgccatgatctggccctattaatccagaagggtctgatggaagcctctgtgattctcttccatggttaaacattttaattgtattatacctcggatattcctaaatatttaaaacactggcatggttgaactagacaacctttaagtagtttgttccaaccatgagatttagatttcatgatttaggttttatgatcttaaactgaaacctgttagttttctaccactagtgagatcatggcctctgcttttctcctgggaagtccctcttataatcactctcttcccatgattaaagggctactctgccttcatgttgctacccgctcccctggaaatggagaatcaagcaaggatgcggttttccttccattactacatccatacaagagtaaatcaagaataaaagtccagttaatgaaaagatcactggtcttaatatacttagcaaaattttaaaggcaattaaaagtatatacatagacaatgatcaaaattctaatgaaaagacccggctctcccctaaaagaagaaaaaatcatgtaatgtatatatgcattccataaaaacatacatggggaaaacttcagaagcctaaaaacaaaacatcagtaaaccaagccacacttagaaaaatgaaagctgatttttattttatcatcaacagccattctttagacatgaacatgcatacgtaatattctacgcacacatcacagcttttaacgttagttaataaaggttaaacacacaacatacatccttacaaaaaaagtcaaaatgcaaacttaaaactttaaacaaaagtattactaatttaaaaaaagtttgtgttgggtaccatttgtacaacacagttaatttaaacattttcattttggttgcacatgaaaaaggcggcagtagaaaataaagtcattgagggtttttaaatagcagaataggcagttttgccatgcaggagaagcaatattaaatattagtttcaaaaaaaatccacatttaaaaatatttagttcaagtcacagaatttttctcagtagagaccccaatgcaatgcataattagctgccttagatggcccgtttgaaaggatgatatcccttcagagtgtaactttactgattttggcacagaaaagaagtcttaagaacatgattaaaaaagagggaagaggaacagaggaaagaaataaaagcaagaataaatgagatagtaattgcaatcactaaaaaactgcattctcagtcattgcagaatactgtcttctgtctacagcaggtgcttattccagaattgttattgcagcatggatttaatttgcttggaggtagtctcatcattcaaatgttttgttgtgtacctgagagcatttagaagaccttccacactattaggaggttggtccttaagaactttgatacaacctttcatatcaattttggaagttttagcaaatgctcccactggatgtacgtggtcatagagtattatgacacccaccattaccctcaagcagaatgacactgtctcttcatttgtaaatctgcttctgtattccggtgtttccagcatgactctgcatacactagccattgtgcttaaacaatctgtggtattttctattggtaaatttttattctctgatacaaattttgttgtggcatcactcaaggttttcagcattggagttgcctcagcataaaacaaagacattcgatttgccaattcattatttacttcattttctccttctgccggtacattgttaatcctcatacgactcaatgttcttctataatagctgaaatcattctgtatggcaggatttgtcatcttgagttcatcaaaccggagtgtgaaatgaagaatttctgcaaactgtttagcaagagcctgctctcgctctagatgctgggtgggagaatatggggtacttgttaaggctcccagaagacctcttaatgctgcttctaacctctgagaaaattcgtaaaatttctttaatttgcctactagtggaacaactgcaccccatgccttctcttgcaacttctcatctgctggatgctggattgcctctcgtatttcgtggccagctcctctgtatgactgcaagtcctccaagatgccttctgcatcttttaatactacattcacctgattataaatttccttctcagactctgtaggctgggcattttcaaagtccaagaaaaaatgtgctgcattgtggtctatgtccctggttagcaccttaatgagattacccatgccagcaaaccttcagccagtgctggtgattctgtccttgtccttctatccttggattggcgttccctctttcctagttcacttgttccagtccttcaacttctgtttcttgctaacaggtgtgcaaatgaattaccttcgagaagccgagccgccggcgctcgcacaaaaggaggacgctcgcctcgcgacgcgcctccccccgcgcccagtccccgccgcatcgc

SEQ ID NO: 18514 - RNA, 3229 nt, Homo sapiens
  source 1..3229: mol_type = other RNA
tgagctgctgtaccaaaataccacaaactgcatggcttaaaacaacagaaatttattccctcacaatcctggaggccagatgtctgaaatcaagatattggtagggttggttccttctcgagactctgagggagaatctgtgacatgcctgttttcctagcttctagtgacttcctccaattcttagggttctttggctcatagatgcattgctctaatctctgcctccatcttcccatggccttcagctctgtgtgtctatttccccttcttttctaagagctagtcattgaatttagggcccaccctactacaggttgatctcatttccaggtccttgatttcatctgcaaaaactttttccaaataatgtcacacgtggagattcccagtgaatgtatctcctgggggccactattcagcctattacactattcttagaagatgcctagaaggatatggccaatgttatccagaaggcttcatgaaggaggtaatagaagctaacccttcaaagatgaaagttggcgttcattagagggtcacaaggggaggaagggaatgtcaggttcagggaccagccagaccagagctaaggaagtgacatcacatggaacaatttgtgaacagcaagcagtagggcctggctgcaggacagggtgtgaagtgggggagcagtgatcaggagggccagagagatcagcagggatgtgatcttgagaagctgtgtgtgccatgatctggccctattaatccagaagggtctgatggaagcctctgtgattctcttccatggttaaacattttaattgtattatacctcggatattcctaaatatttaaaacactggcatggttgaactagacaacctttaagtagtttgttccaaccatgagatttagatttcatgatttaggttttatgatcttaaactgaaacctgttagttttctaccactagtgagatcatggcctctgcttttctcctgggaagtccctcttataatcactctcttcccatgattaaagggctactctgccttcatgttgctacccgctcccctggaaatggagaatcaagcaaggatgcggttttccttccattactacatccatacaagagtaaatcaagaataaaagtccagttaatgaaaagatcactggtcttaatatacttagcaaaattttaaaggcaattaaaagtatatacatagacaatgatcaaaattctaatgaaaagacccggctctcccctaaaagaagaaaaaatcatgtaatgtatatatgcattccataaaaacatacatggggaaaacttcagaagcctaaaaacaaaacatcagtaaaccaagccacacttagaaaaatgaaagctgatttttattttatcatcaacagccattctttagacatgaacatgcatacgtaatattctacgcacacatcacagcttttaacgttagttaataaaggttaaacacacaacatacatccttacaaaaaaagtcaaaatgcaaacttaaaactttaaacaaaagtattactaatttaaaaaaagtttgtgttgggtaccatttgtacaacacagttaatttaaacattttcattttggttgcacatgaaaaaggcggcagtagaaaataaagtcattgagggtttttaaatagcagaataggcagttttgccatgcaggagaagcaatattaaatattagtttcaaaaaaaatccacatttaaaaatatttagttcaagtcacagaatttttctcagtagagaccccaatgcaatgcataattagctgccttagatggcccgtttgaaaggatgatatcccttcagagtgtaactttactgattttggcacagaaaagaagtcttaagaacatgattaaaaaagagggaagaggaacagaggaaagaaataaaagcaagaataaatgagatagtaattgcaatcactaaaaaactgcattctcagtcattgcagaatactgtcttctgtctacagcaggtgcttattccagaattgttattgcagcatggatttaatttgcttggaggtagtctcatcattcaaatgttttgttgtgtacctgagagcatttagaagaccttccacactattaggaggttggtccttaagaactttgatacaacctttcatatcaattttggaagttttagcaaatgctcccactggatgtacgtggtcatagagtattatgacacccaccattaccctcaagcagaatgacactgtctcttcatttgtaaatctgcttctgtattccggtgtttccagcatgactctgcatacactagccattgtgcttaaacaatctgtggtattttctattggtaaatttttattctctgatacaaattttgttgtggcatcactcaaggttttcagcattggagttgcctcagcataaaacaaagacattcgatttgccaattcattatttacttcattttctccttctgccggtacattgttaatcctcatacgactcaatgttcttctataatagctgaaatcattctgtatggcaggatttgtcatcttgagttcatcaaaccggagtgtgaaatgaagaatttctgcaaactgtttagcaagagcctgctctcgctctagatgctgggtgggagaatatggggtacttgttaaggctcccagaagacctcttaatgctgcttctaacctctgagaaaattcgtaaaatttctttaatttgcctactagtggaacaactgcaccccatgccttctcttgcaacttctcatctgctggatgctggattgcctctcgtatttcgtggccagctcctctgtatgactgcaagtcctccaagatgccttctgcatcttttaatactacattcacctgattataaatttccttctcagactctgtaggctgggcattttcaaagtccaagaaaaaatgtgctgcattgtggtctatgtccctggttagcaccttaatgagattacccatgccagcaaaccttcagccagtgctggtgattctgtccttgtccttctatctgtttaaggaaagaaaaaaaggaagaaagtcaactgggtaaccttgaatgagttaatcaaattccaggcctcagtttcttctccttcgagaagccgagccgccggcgctcgcacaaaaggaggacgctcgcctcgcgacgcgcctccccccgcgcccagtccccgccgcatcgc

SEQ ID NO: 18515 - RNA, 3145 nt, Homo sapiens
  source 1..3145: mol_type = other RNA
tgagctgctgtaccaaaataccacaaactgcatggcttaaaacaacagaaatttattccctcacaatcctggaggccagatgtctgaaatcaagatattggtagggttggttccttctcgagactctgagggagaatctgtgacatgcctgttttcctagcttctagtgacttcctccaattcttagggttctttggctcatagatgcattgctctaatctctgcctccatcttcccatggccttcagctctgtgtgtctatttccccttcttttctaagagctagtcattgaatttagggcccaccctactacaggttgatctcatttccaggtccttgatttcatctgcaaaaactttttccaaataatgtcacacgtggagattcccagtgaatgtatctcctgggggccactattcagcctattacactattcttagaagatgcctagaaggatatggccaatgttatccagaaggcttcatgaaggaggtaatagaagctaacccttcaaagatgaaagttggcgttcattagagggtcacaaggggaggaagggaatgtcaggttcagggaccagccagaccagagctaaggaagtgacatcacatggaacaatttgtgaacagcaagcagtagggcctggctgcaggacagggtgtgaagtgggggagcagtgatcaggagggccagagagatcagcagggatgtgatcttgagaagctgtgtgtgccatgatctggccctattaatccagaagggtctgatggaagcctctgtgattctcttccatggttaaacattttaattgtattatacctcggatattcctaaatatttaaaacactggcatggttgaactagacaacctttaagtagtttgttccaaccatgagatttagatttcatgatttaggttttatgatcttaaactgaaacctgttagttttctaccactagtgagatcatggcctctgcttttctcctgggaagtccctcttataatcactctcttcccatgattaaagggctactctgccttcatgttgctacccgctcccctggaaatggagaatcaagcaaggatgcggttttccttccattactacatccatacaagagtaaatcaagaataaaagtccagttaatgaaaagatcactggtcttaatatacttagcaaaattttaaaggcaattaaaagtatatacatagacaatgatcaaaattctaatgaaaagacccggctctcccctaaaagaagaaaaaatcatgtaatgtatatatgcattccataaaaacatacatggggaaaacttcagaagcctaaaaacaaaacatcagtaaaccaagccacacttagaaaaatgaaagctgatttttattttatcatcaacagccattctttagacatgaacatgcatacgtaatattctacgcacacatcacagcttttaacgttagttaataaaggttaaacacacaacatacatccttacaaaaaaagtcaaaatgcaaacttaaaactttaaacaaaagtattactaatttaaaaaaagtttgtgttgggtaccatttgtacaacacagttaatttaaacattttcattttggttgcacatgaaaaaggcggcagtagaaaataaagtcattgagggtttttaaatagcagaataggcagttttgccatgcaggagaagcaatattaaatattagtttcaaaaaaaatccacatttaaaaatatttagttcaagtcacagaatttttctcagtagagaccccaatgcaatgcataattagctgccttagatggcccgtttgaaaggatgatatcccttcagagtgtaactttactgattttggcacagaaaagaagtcttaagaacatgattaaaaaagagggaagaggaacagaggaaagaaataaaagcaagaataaatgagatagtaattgcaatcactaaaaaactgcattctcagtcattgcagaatactgtcttctgtctacagcaggtgcttattccagaattgttattgcagcatggatttaatttgcttggaggtagtctcatcattcaaatgttttgttgtgtacctgagagcatttagaagaccttccacactattaggaggttggtccttaagaactttgatacaacctttcatatcaattttggaagttttagcaaatgctcccactggatgtacgtggtcatagagtattatgacacccaccattaccctcaagcagaatgacactgtctcttcatttgtaaatctgcttctgtattccggtgtttccagcatgactctgcatacactagccattgtgcttaaacaatctgtggtattttctattggtaaatttttattctctgatacaaattttgttgtggcatcactcaaggttttcagcattggagttgcctcagcataaaacaaagacattcgatttgccaattcattatttacttcattttctccttctgccggtacattgttaatcctcatacgactcaatgttcttctataatagctgaaatcattctgtatggcaggatttgtcatcttgagttcatcaaaccggagtgtgaaatgaagaatttctgcaaactgtttagcaagagcctgctctcgctctagatgctgggtgggagaatatggggtacttgttaaggctcccagaagacctcttaatgctgcttctaacctctgagaaaattcgtaaaatttctttaatttgcctactagtggaacaactgcaccccatgccttctcttgcaacttctcatctgctggatgctggattgcctctcgtatttcgtggccagctcctctgtatgactgcaagtcctccaagatgccttctgcatcttttaatactacattcacctgattataaatttccttctcagactctgtaggctgggcattttcaaagtccaagaaaaaatgtgctgcattgtggtctatgtccctggttagcaccttaatgagattacccatgccagcaaaccttcagccagtgctggtgattctgtccttgtccttctatcttcgagaagccgagccgccggcgctcgcacaaaaggaggacgctcgcctcgcgacgcgcctccccccgcgcccagtccccgccgcatcgc

SEQ ID NO: 18516 - RNA, 3391 nt, Homo sapiens
  source 1..3391: mol_type = other RNA
tgagctgctgtaccaaaataccacaaactgcatggcttaaaacaacagaaatttattccctcacaatcctggaggccagatgtctgaaatcaagatattggtagggttggttccttctcgagactctgagggagaatctgtgacatgcctgttttcctagcttctagtgacttcctccaattcttagggttctttggctcatagatgcattgctctaatctctgcctccatcttcccatggccttcagctctgtgtgtctatttccccttcttttctaagagctagtcattgaatttagggcccaccctactacaggttgatctcatttccaggtccttgatttcatctgcaaaaactttttccaaataatgtcacacgtggagattcccagtgaatgtatctcctgggggccactattcagcctattacactattcttagaagatgcctagaaggatatggccaatgttatccagaaggcttcatgaaggaggtaatagaagctaacccttcaaagatgaaagttggcgttcattagagggtcacaaggggaggaagggaatgtcaggttcagggaccagccagaccagagctaaggaagtgacatcacatggaacaatttgtgaacagcaagcagtagggcctggctgcaggacagggtgtgaagtgggggagcagtgatcaggagggccagagagatcagcagggatgtgatcttgagaagctgtgtgtgccatgatctggccctattaatccagaagggtctgatggaagcctctgtgattctcttccatggttaaacattttaattgtattatacctcggatattcctaaatatttaaaacactggcatggttgaactagacaacctttaagtagtttgttccaaccatgagatttagatttcatgatttaggttttatgatcttaaactgaaacctgttagttttctaccactagtgagatcatggcctctgcttttctcctgggaagtccctcttataatcactctcttcccatgattaaagggctactctgccttcatgttgctacccgctcccctggaaatggagaatcaagcaaggatgcggttttccttccattactacatccatacaagagtaaatcaagaataaaagtccagttaatgaaaagatcactggtcttaatatacttagcaaaattttaaaggcaattaaaagtatatacatagacaatgatcaaaattctaatgaaaagacccggctctcccctaaaagaagaaaaaatcatgtaatgtatatatgcattccataaaaacatacatggggaaaacttcagaagcctaaaaacaaaacatcagtaaaccaagccacacttagaaaaatgaaagctgatttttattttatcatcaacagccattctttagacatgaacatgcatacgtaatattctacgcacacatcacagcttttaacgttagttaataaaggttaaacacacaacatacatccttacaaaaaaagtcaaaatgcaaacttaaaactttaaacaaaagtattactaatttaaaaaaagtttgtgttgggtaccatttgtacaacacagttaatttaaacattttcattttggttgcacatgaaaaaggcggcagtagaaaataaagtcattgagggtttttaaatagcagaataggcagttttgccatgcaggagaagcaatattaaatattagtttcaaaaaaaatccacatttaaaaatatttagttcaagtcacagaatttttctcagtagagaccccaatgcaatgcataattagctgccttagatggcccgtttgaaaggatgatatcccttcagagtgtaactttactgattttggcacagaaaagaagtcttaagaacatgattaaaaaagagggaagaggaacagaggaaagaaataaaagcaagaataaatgagatagtaattgcaatcactaaaaaactgcattctcagtcattgcagaatactgtcttctgtctacagcaggtgcttattccagaattgttattgcagcatggatttaatttgcttggaggtagtctcatcattcaaatgttttgttgtgtacctgagagcatttagaagaccttccacactattaggaggttggtccttaagaactttgatacaacctttcatatcaattttggaagttttagcaaatgctcccactggatgtacgtggtcatagagtattatgacacccaccattaccctcaagcagaatgacactgtctcttcatttgtaaatctgcttctgtattccggtgtttccagcatgactctgcatacactagccattgtgcttaaacaatctgtggtattttctattggtaaatttttattctctgatacaaattttgttgtggcatcactcaaggttttcagcattggagttgcctcagcataaaacaaagacattcgatttgccaattcattatttacttcattttctccttctgccggtacattgttaatcctcatacgactcaatgttcttctataatagctgaaatcattctgtatggcaggatttgtcatcttgagttcatcaaaccggagtgtgaaatgaagaatttctgcaaactgtttagcaagagcctgctctcgctctagatgctgggtgggagaatatggggtacttgttaaggctcccagaagacctcttaatgctgcttctaacctctgagaaaattcgtaaaatttctttaatttgcctactagtggaacaactgcaccccatgccttctcttgcaacttctcatctgctggatgctggattgcctctcgtatttcgtggccagctcctctgtatgactgcaagtcctccaagatgccttctgcatcttttaatactacattcacctgattataaatttccttctcagactctgtaggctgggcattttcaaagtccaagaaaaaatgtgctgcattgtggtctatgtccctggttagcaccttaatgagattacccatgccagcaaactgccaagtaaacaggccttgtggcagtgaaaggataaactgtccatcattctttcttctcctcggagatttcacaggaaaaggagaaagcgcaggaaacaggaggccttcagccagtgctggtgattctgtccttgtccttctatccttggattggcgttccctctttcctagttcacttgttccagtccttcaacttctgtttcttgctaacaggtgtgcaaatgaattaccaactgggtaaccttgaatgagttaatcaaattccaggcctcagtttcttctccttcgagaagccgagccgccggcgctcgcacaaaaggaggacgctcgcctcgcgacgcgcctccccccgcgcccagtccccgccgcatcgc

SEQ ID NO: 18517 - RNA, 3030 nt, Homo sapiens
  source 1..3030: mol_type = other RNA
tgagctgctgtaccaaaataccacaaactgcatggcttaaaacaacagaaatttattccctcacaatcctggaggccagatgtctgaaatcaagatattggtagggttggttccttctcgagactctgagggagaatctgtgacatgcctgttttcctagcttctagtgacttcctccaattcttagggttctttggctcatagatgcattgctctaatctctgcctccatcttcccatggccttcagctctgtgtgtctatttccccttcttttctaagagctagtcattgaatttagggcccaccctactacaggttgatctcatttccaggtccttgatttcatctgcaaaaactttttccaaataatgtcacacgtggagattcccagtgaatgtatctcctgggggccactattcagcctattacactattcttagaagatgcctagaaggatatggccaatgttatccagaaggcttcatgaaggaggtaatagaagctaacccttcaaagatgaaagttggcgttcattagagggtcacaaggggaggaagggaatgtcaggttcagggaccagccagaccagagctaaggaagtgacatcacatggaacaatttgtgaacagcaagcagtagggcctggctgcaggacagggtgtgaagtgggggagcagtgatcaggagggccagagagatcagcagggatgtgatcttgagaagctgtgtgtgccatgatctggccctattaatccagaagggtctgatggaagcctctgtgattctcttccatggttaaacattttaattgtattatacctcggatattcctaaatatttaaaacactggcatggttgaactagacaacctttaagtagtttgttccaaccatgagatttagatttcatgatttaggttttatgatcttaaactgaaacctgttagttttctaccactagtgagatcatggcctctgcttttctcctgggaagtccctcttataatcactctcttcccatgattaaagggctactctgccttcatgttgctacccgctcccctggaaatggagaatcaagcaaggatgcggttttccttccattactacatccatacaagagtaaatcaagaataaaagtccagttaatgaaaagatcactggtcttaatatacttagcaaaattttaaaggcaattaaaagtatatacatagacaatgatcaaaattctaatgaaaagacccggctctcccctaaaagaagaaaaaatcatgtaatgtatatatgcattccataaaaacatacatggggaaaacttcagaagcctaaaaacaaaacatcagtaaaccaagccacacttagaaaaatgaaagctgatttttattttatcatcaacagccattctttagacatgaacatgcatacgtaatattctacgcacacatcacagcttttaacgttagttaataaaggttaaacacacaacatacatccttacaaaaaaagtcaaaatgcaaacttaaaactttaaacaaaagtattactaatttaaaaaaagtttgtgttgggtaccatttgtacaacacagttaatttaaacattttcattttggttgcacatgaaaaaggcggcagtagaaaataaagtcattgagggtttttaaatagcagaataggcagttttgccatgcaggagaagcaatattaaatattagtttcaaaaaaaatccacatttaaaaatatttagttcaagtcacagaatttttctcagtagagaccccaatgcaatgcataattagctgccttagatggcccgtttgaaaggatgatatcccttcagagtgtaactttactgattttggcacagaaaagaagtcttaagaacatgattaaaaaagagggaagaggaacagaggaaagaaataaaagcaagaataaatgagatagtaattgcaatcactaaaaaactgcattctcagtcattgcagaatactgtcttctgtctacagcaggtgcttattccagaattgttattgcagcatggatttaatttgcttggaggtagtctcatcattcaaatgttttgttgtgtacctgagagcatttagaagaccttccacactattaggaggttggtccttaagaactttgatacaacctttcatatcaattttggaagttttagcaaatgctcccactggatgtacgtggtcatagagtattatgacacccaccattaccctcaagcagaatgacactgtctcttcatttgtaaatctgcttctgtattccggtgtttccagcatgactctgcatacactagccattgtgcttaaacaatctgtggtattttctattggtaaatttttattctctgatacaaattttgttgtggcatcactcaaggttttcagcattggagttgcctcagcataaaacaaagacattcgatttgccaattcattatttacttcattttctccttctgccggtacattgttaatcctcatacgactcaatgttcttctataatagctgaaatcattctgtatggcaggatttgtcatcttgagttcatcaaaccggagtgtgaaatgaagaatttctgcaaactgtttagcaagagcctgctctcgctctagatgctgggtgggagaatatggggtacttgttaaggctcccagaagacctcttaatgctgcttctctcgtatttcgtggccagctcctctgtatgactgcaagtcctccaagatgccttctgcatcttttaatactacattcacctgattataaatttccttctcagactctgtaggctgggcatcttcagccagtgctggtgattctgtccttgtccttctatcaactgggtaaccttgaatgagttaatcaaattccaggcctcagtttcttctcctggacttcaggaatggtgacagcccctgcctggctcacctcgcagcggggtcagtgagaggaatgctgtccacgcacccattcagccctcccgcagatacttactgggcct

SEQ ID NO: 18518 - RNA, 3109 nt, Homo sapiens
  source 1..3109: mol_type = other RNA
tgagctgctgtaccaaaataccacaaactgcatggcttaaaacaacagaaatttattccctcacaatcctggaggccagatgtctgaaatcaagatattggtagggttggttccttctcgagactctgagggagaatctgtgacatgcctgttttcctagcttctagtgacttcctccaattcttagggttctttggctcatagatgcattgctctaatctctgcctccatcttcccatggccttcagctctgtgtgtctatttccccttcttttctaagagctagtcattgaatttagggcccaccctactacaggttgatctcatttccaggtccttgatttcatctgcaaaaactttttccaaataatgtcacacgtggagattcccagtgaatgtatctcctgggggccactattcagcctattacactattcttagaagatgcctagaaggatatggccaatgttatccagaaggcttcatgaaggaggtaatagaagctaacccttcaaagatgaaagttggcgttcattagagggtcacaaggggaggaagggaatgtcaggttcagggaccagccagaccagagctaaggaagtgacatcacatggaacaatttgtgaacagcaagcagtagggcctggctgcaggacagggtgtgaagtgggggagcagtgatcaggagggccagagagatcagcagggatgtgatcttgagaagctgtgtgtgccatgatctggccctattaatccagaagggtctgatggaagcctctgtgattctcttccatggttaaacattttaattgtattatacctcggatattcctaaatatttaaaacactggcatggttgaactagacaacctttaagtagtttgttccaaccatgagatttagatttcatgatttaggttttatgatcttaaactgaaacctgttagttttctaccactagtgagatcatggcctctgcttttctcctgggaagtccctcttataatcactctcttcccatgattaaagggctactctgccttcatgttgctacccgctcccctggaaatggagaatcaagcaaggatgcggttttccttccattactacatccatacaagagtaaatcaagaataaaagtccagttaatgaaaagatcactggtcttaatatacttagcaaaattttaaaggcaattaaaagtatatacatagacaatgatcaaaattctaatgaaaagacccggctctcccctaaaagaagaaaaaatcatgtaatgtatatatgcattccataaaaacatacatggggaaaacttcagaagcctaaaaacaaaacatcagtaaaccaagccacacttagaaaaatgaaagctgatttttattttatcatcaacagccattctttagacatgaacatgcatacgtaatattctacgcacacatcacagcttttaacgttagttaataaaggttaaacacacaacatacatccttacaaaaaaagtcaaaatgcaaacttaaaactttaaacaaaagtattactaatttaaaaaaagtttgtgttgggtaccatttgtacaacacagttaatttaaacattttcattttggttgcacatgaaaaaggcggcagtagaaaataaagtcattgagggtttttaaatagcagaataggcagttttgccatgcaggagaagcaatattaaatattagtttcaaaaaaaatccacatttaaaaatatttagttcaagtcacagaatttttctcagtagagaccccaatgcaatgcataattagctgccttagatggcccgtttgaaaggatgatatcccttcagagtgtaactttactgattttggcacagaaaagaagtcttaagaacatgattaaaaaagagggaagaggaacagaggaaagaaataaaagcaagaataaatgagatagtaattgcaatcactaaaaaactgcattctcagtcattgcagaatactgtcttctgtctacagcaggtgcttattccagaattgttattgcagcatggatttaatttgcttggaggtagtctcatcattcaaatgttttgttgtgtacctgagagcatttagaagaccttccacactattaggaggttggtccttaagaactttgatacaacctttcatatcaattttggaagttttagcaaatgctcccactggatgtacgtggtcatagagtattatgacacccaccattaccctcaagcagaatgacactgtctcttcatttgtaaatctgcttctgtattccggtgtttccagcatgactctgcatacactagccattgtgcttaaacaatctgtggtattttctattggtaaatttttattctctgatacaaattttgttgtggcatcactcaaggttttcagcattggagttgcctcagcataaaacaaagacattcgatttgccaattcattatttacttcattttctccttctgccggtacattgttaatcctcatacgactcaatgttcttctataatagctgaaatcattctgtatggcaggatttgtcatcttgagttcatcaaaccggagtgtgaaatgaagaatttctgcaaactgtttagcaagagcctgctctcgctctagatgctgggtgggagaatatggggtacttgttaaggctcccagaagacctcttaatgctgcttctctcgtatttcgtggccagctcctctgtatgactgcaagtcctccaagatgccttctgcatcttttaatactacattcacctgattataaatttccttctcagactctgtaggctgggcatcttcagccagtgctggtgattctgtccttgtccttctatcaactgggtaaccttgaatgagttaatcaaattccaggcctcagtttcttctcctggcggcccgggcgggcgaggggagcgcggcgcgggagcgcaggagcctcggagcctccggtgccgccgccgccgccgtttccgggttggcggggctcacgtcaccgccacaggtttgcgagctgcccccgccgcggcggcagcagcagcagcagcagcagcccgggcgagtgccaggcgagaaataact

SEQ ID NO: 18519 - RNA, 3069 nt, Homo sapiens
  source 1..3069: mol_type = other RNA
tgagctgctgtaccaaaataccacaaactgcatggcttaaaacaacagaaatttattccctcacaatcctggaggccagatgtctgaaatcaagatattggtagggttggttccttctcgagactctgagggagaatctgtgacatgcctgttttcctagcttctagtgacttcctccaattcttagggttctttggctcatagatgcattgctctaatctctgcctccatcttcccatggccttcagctctgtgtgtctatttccccttcttttctaagagctagtcattgaatttagggcccaccctactacaggttgatctcatttccaggtccttgatttcatctgcaaaaactttttccaaataatgtcacacgtggagattcccagtgaatgtatctcctgggggccactattcagcctattacactattcttagaagatgcctagaaggatatggccaatgttatccagaaggcttcatgaaggaggtaatagaagctaacccttcaaagatgaaagttggcgttcattagagggtcacaaggggaggaagggaatgtcaggttcagggaccagccagaccagagctaaggaagtgacatcacatggaacaatttgtgaacagcaagcagtagggcctggctgcaggacagggtgtgaagtgggggagcagtgatcaggagggccagagagatcagcagggatgtgatcttgagaagctgtgtgtgccatgatctggccctattaatccagaagggtctgatggaagcctctgtgattctcttccatggttaaacattttaattgtattatacctcggatattcctaaatatttaaaacactggcatggttgaactagacaacctttaagtagtttgttccaaccatgagatttagatttcatgatttaggttttatgatcttaaactgaaacctgttagttttctaccactagtgagatcatggcctctgcttttctcctgggaagtccctcttataatcactctcttcccatgattaaagggctactctgccttcatgttgctacccgctcccctggaaatggagaatcaagcaaggatgcggttttccttccattactacatccatacaagagtaaatcaagaataaaagtccagttaatgaaaagatcactggtcttaatatacttagcaaaattttaaaggcaattaaaagtatatacatagacaatgatcaaaattctaatgaaaagacccggctctcccctaaaagaagaaaaaatcatgtaatgtatatatgcattccataaaaacatacatggggaaaacttcagaagcctaaaaacaaaacatcagtaaaccaagccacacttagaaaaatgaaagctgatttttattttatcatcaacagccattctttagacatgaacatgcatacgtaatattctacgcacacatcacagcttttaacgttagttaataaaggttaaacacacaacatacatccttacaaaaaaagtcaaaatgcaaacttaaaactttaaacaaaagtattactaatttaaaaaaagtttgtgttgggtaccatttgtacaacacagttaatttaaacattttcattttggttgcacatgaaaaaggcggcagtagaaaataaagtcattgagggtttttaaatagcagaataggcagttttgccatgcaggagaagcaatattaaatattagtttcaaaaaaaatccacatttaaaaatatttagttcaagtcacagaatttttctcagtagagaccccaatgcaatgcataattagctgccttagatggcccgtttgaaaggatgatatcccttcagagtgtaactttactgattttggcacagaaaagaagtcttaagaacatgattaaaaaagagggaagaggaacagaggaaagaaataaaagcaagaataaatgagatagtaattgcaatcactaaaaaactgcattctcagtcattgcagaatactgtcttctgtctacagcaggtgcttattccagaattgttattgcagcatggatttaatttgcttggaggtagtctcatcattcaaatgttttgttgtgtacctgagagcatttagaagaccttccacactattaggaggttggtccttaagaactttgatacaacctttcatatcaattttggaagttttagcaaatgctcccactggatgtacgtggtcatagagtattatgacacccaccattaccctcaagcagaatgacactgtctcttcatttgtaaatctgcttctgtattccggtgtttccagcatgactctgcatacactagccattgtgcttaaacaatctgtggtattttctattggtaaatttttattctctgatacaaattttgttgtggcatcactcaaggttttcagcattggagttgcctcagcataaaacaaagacattcgatttgccaattcattatttacttcattttctccttctgccggtacattgttaatcctcatacgactcaatgttcttctataatagctgaaatcattctgtatggcaggatttgtcatcttgagttcatcaaaccggagtgtgaaatgaagaatttctgcaaactgtttagcaagagcctgctctcgctctagatgctgggtgggagaatatggggtacttgttaaggctcccagaagacctcttaatgctgcttctctcgtatttcgtggccagctcctctgtatgactgcaagtcctccaagatgccttctgcatcttttaatactacattcacctgattataaatttccttctcagactctgtaggctgggcatcttcagccagtgctggtgattctgtccttgtccttctatcctccgctcgagcctccaggcgctctcagtcccgctcctgcgccctcctggagccgcagaggcggctcctcagcggcgctagggggagccccgggtccggagcgggggagcggcggcagccggaccgggagcccctcaacacctgcccctgtggcagagccgcgacaagccaggcggcagctccgagcggggagggcaagtgac

SEQ ID NO: 18520 - RNA, 3196 nt, Homo sapiens
  source 1..3196: mol_type = other RNA
tgagctgctgtaccaaaataccacaaactgcatggcttaaaacaacagaaatttattccctcacaatcctggaggccagatgtctgaaatcaagatattggtagggttggttccttctcgagactctgagggagaatctgtgacatgcctgttttcctagcttctagtgacttcctccaattcttagggttctttggctcatagatgcattgctctaatctctgcctccatcttcccatggccttcagctctgtgtgtctatttccccttcttttctaagagctagtcattgaatttagggcccaccctactacaggttgatctcatttccaggtccttgatttcatctgcaaaaactttttccaaataatgtcacacgtggagattcccagtgaatgtatctcctgggggccactattcagcctattacactattcttagaagatgcctagaaggatatggccaatgttatccagaaggcttcatgaaggaggtaatagaagctaacccttcaaagatgaaagttggcgttcattagagggtcacaaggggaggaagggaatgtcaggttcagggaccagccagaccagagctaaggaagtgacatcacatggaacaatttgtgaacagcaagcagtagggcctggctgcaggacagggtgtgaagtgggggagcagtgatcaggagggccagagagatcagcagggatgtgatcttgagaagctgtgtgtgccatgatctggccctattaatccagaagggtctgatggaagcctctgtgattctcttccatggttaaacattttaattgtattatacctcggatattcctaaatatttaaaacactggcatggttgaactagacaacctttaagtagtttgttccaaccatgagatttagatttcatgatttaggttttatgatcttaaactgaaacctgttagttttctaccactagtgagatcatggcctctgcttttctcctgggaagtccctcttataatcactctcttcccatgattaaagggctactctgccttcatgttgctacccgctcccctggaaatggagaatcaagcaaggatgcggttttccttccattactacatccatacaagagtaaatcaagaataaaagtccagttaatgaaaagatcactggtcttaatatacttagcaaaattttaaaggcaattaaaagtatatacatagacaatgatcaaaattctaatgaaaagacccggctctcccctaaaagaagaaaaaatcatgtaatgtatatatgcattccataaaaacatacatggggaaaacttcagaagcctaaaaacaaaacatcagtaaaccaagccacacttagaaaaatgaaagctgatttttattttatcatcaacagccattctttagacatgaacatgcatacgtaatattctacgcacacatcacagcttttaacgttagttaataaaggttaaacacacaacatacatccttacaaaaaaagtcaaaatgcaaacttaaaactttaaacaaaagtattactaatttaaaaaaagtttgtgttgggtaccatttgtacaacacagttaatttaaacattttcattttggttgcacatgaaaaaggcggcagtagaaaataaagtcattgagggtttttaaatagcagaataggcagttttgccatgcaggagaagcaatattaaatattagtttcaaaaaaaatccacatttaaaaatatttagttcaagtcacagaatttttctcagtagagaccccaatgcaatgcataattagctgccttagatggcccgtttgaaaggatgatatcccttcagagtgtaactttactgattttggcacagaaaagaagtcttaagaacatgattaaaaaagagggaagaggaacagaggaaagaaataaaagcaagaataaatgagatagtaattgcaatcactaaaaaactgcattctcagtcattgcagaatactgtcttctgtctacagcaggtgcttattccagaattgttattgcagcatggatttaatttgcttggaggtagtctcatcattcaaatgttttgttgtgtacctgagagcatttagaagaccttccacactattaggaggttggtccttaagaactttgatacaacctttcatatcaattttggaagttttagcaaatgctcccactggatgtacgtggtcatagagtattatgacacccaccattaccctcaagcagaatgacactgtctcttcatttgtaaatctgcttctgtattccggtgtttccagcatgactctgcatacactagccattgtgcttaaacaatctgtggtattttctattggtaaatttttattctctgatacaaattttgttgtggcatcactcaaggttttcagcattggagttgcctcagcataaaacaaagacattcgatttgccaattcattatttacttcattttctccttctgccggtacattgttaatcctcatacgactcaatgttcttctataatagctgaaatcattctgtatggcaggatttgtcatcttgagttcatcaaaccggagtgtgaaatgaagaatttctgcaaactgtttagcaagagcctgctctcgctctagatgctgggtgggagaatatggggtacttgttaaggctcccagaagacctcttaatgctgcttctctcgtatttcgtggccagctcctctgtatgactgcaagtcctccaagatgccttctgcatcttttaatactacattcacctgattataaatttccttctcagactctgtaggctgggcatcttcagccagtgctggtgattctgtccttgtccttctatccttggattggcgttccctctttcctagttcacttgttccagtccttcaacttctgtttcttgctaacaggtgtgcaaatgaattaccaactgggtaaccttgaatgagttaatcaaattccaggcctcagtttcttctcctggcggcccgggcgggcgaggggagcgcggcgcgggagcgcaggagcctcggagcctccggtgccgccgccgccgccgtttccgggttggcggggctcacgtcaccgccacaggtttgcgagctgcccccgccgcggcggcagcagcagcagcagcagcagcccgggcgagtgccaggcgagaaataact

SEQ ID NO: 18521 - RNA, 3156 nt, Homo sapiens
  source 1..3156: mol_type = other RNA
tgagctgctgtaccaaaataccacaaactgcatggcttaaaacaacagaaatttattccctcacaatcctggaggccagatgtctgaaatcaagatattggtagggttggttccttctcgagactctgagggagaatctgtgacatgcctgttttcctagcttctagtgacttcctccaattcttagggttctttggctcatagatgcattgctctaatctctgcctccatcttcccatggccttcagctctgtgtgtctatttccccttcttttctaagagctagtcattgaatttagggcccaccctactacaggttgatctcatttccaggtccttgatttcatctgcaaaaactttttccaaataatgtcacacgtggagattcccagtgaatgtatctcctgggggccactattcagcctattacactattcttagaagatgcctagaaggatatggccaatgttatccagaaggcttcatgaaggaggtaatagaagctaacccttcaaagatgaaagttggcgttcattagagggtcacaaggggaggaagggaatgtcaggttcagggaccagccagaccagagctaaggaagtgacatcacatggaacaatttgtgaacagcaagcagtagggcctggctgcaggacagggtgtgaagtgggggagcagtgatcaggagggccagagagatcagcagggatgtgatcttgagaagctgtgtgtgccatgatctggccctattaatccagaagggtctgatggaagcctctgtgattctcttccatggttaaacattttaattgtattatacctcggatattcctaaatatttaaaacactggcatggttgaactagacaacctttaagtagtttgttccaaccatgagatttagatttcatgatttaggttttatgatcttaaactgaaacctgttagttttctaccactagtgagatcatggcctctgcttttctcctgggaagtccctcttataatcactctcttcccatgattaaagggctactctgccttcatgttgctacccgctcccctggaaatggagaatcaagcaaggatgcggttttccttccattactacatccatacaagagtaaatcaagaataaaagtccagttaatgaaaagatcactggtcttaatatacttagcaaaattttaaaggcaattaaaagtatatacatagacaatgatcaaaattctaatgaaaagacccggctctcccctaaaagaagaaaaaatcatgtaatgtatatatgcattccataaaaacatacatggggaaaacttcagaagcctaaaaacaaaacatcagtaaaccaagccacacttagaaaaatgaaagctgatttttattttatcatcaacagccattctttagacatgaacatgcatacgtaatattctacgcacacatcacagcttttaacgttagttaataaaggttaaacacacaacatacatccttacaaaaaaagtcaaaatgcaaacttaaaactttaaacaaaagtattactaatttaaaaaaagtttgtgttgggtaccatttgtacaacacagttaatttaaacattttcattttggttgcacatgaaaaaggcggcagtagaaaataaagtcattgagggtttttaaatagcagaataggcagttttgccatgcaggagaagcaatattaaatattagtttcaaaaaaaatccacatttaaaaatatttagttcaagtcacagaatttttctcagtagagaccccaatgcaatgcataattagctgccttagatggcccgtttgaaaggatgatatcccttcagagtgtaactttactgattttggcacagaaaagaagtcttaagaacatgattaaaaaagagggaagaggaacagaggaaagaaataaaagcaagaataaatgagatagtaattgcaatcactaaaaaactgcattctcagtcattgcagaatactgtcttctgtctacagcaggtgcttattccagaattgttattgcagcatggatttaatttgcttggaggtagtctcatcattcaaatgttttgttgtgtacctgagagcatttagaagaccttccacactattaggaggttggtccttaagaactttgatacaacctttcatatcaattttggaagttttagcaaatgctcccactggatgtacgtggtcatagagtattatgacacccaccattaccctcaagcagaatgacactgtctcttcatttgtaaatctgcttctgtattccggtgtttccagcatgactctgcatacactagccattgtgcttaaacaatctgtggtattttctattggtaaatttttattctctgatacaaattttgttgtggcatcactcaaggttttcagcattggagttgcctcagcataaaacaaagacattcgatttgccaattcattatttacttcattttctccttctgccggtacattgttaatcctcatacgactcaatgttcttctataatagctgaaatcattctgtatggcaggatttgtcatcttgagttcatcaaaccggagtgtgaaatgaagaatttctgcaaactgtttagcaagagcctgctctcgctctagatgctgggtgggagaatatggggtacttgttaaggctcccagaagacctcttaatgctgcttctctcgtatttcgtggccagctcctctgtatgactgcaagtcctccaagatgccttctgcatcttttaatactacattcacctgattataaatttccttctcagactctgtaggctgggcatcttcagccagtgctggtgattctgtccttgtccttctatccttggattggcgttccctctttcctagttcacttgttccagtccttcaacttctgtttcttgctaacaggtgtgcaaatgaattaccctccgctcgagcctccaggcgctctcagtcccgctcctgcgccctcctggagccgcagaggcggctcctcagcggcgctagggggagccccgggtccggagcgggggagcggcggcagccggaccgggagcccctcaacacctgcccctgtggcagagccgcgacaagccaggcggcagctccgagcggggagggcaagtgac

SEQ ID NO: 18522 - RNA, 3192 nt, Homo sapiens
  source 1..3192: mol_type = other RNA
tgagctgctgtaccaaaataccacaaactgcatggcttaaaacaacagaaatttattccctcacaatcctggaggccagatgtctgaaatcaagatattggtagggttggttccttctcgagactctgagggagaatctgtgacatgcctgttttcctagcttctagtgacttcctccaattcttagggttctttggctcatagatgcattgctctaatctctgcctccatcttcccatggccttcagctctgtgtgtctatttccccttcttttctaagagctagtcattgaatttagggcccaccctactacaggttgatctcatttccaggtccttgatttcatctgcaaaaactttttccaaataatgtcacacgtggagattcccagtgaatgtatctcctgggggccactattcagcctattacactattcttagaagatgcctagaaggatatggccaatgttatccagaaggcttcatgaaggaggtaatagaagctaacccttcaaagatgaaagttggcgttcattagagggtcacaaggggaggaagggaatgtcaggttcagggaccagccagaccagagctaaggaagtgacatcacatggaacaatttgtgaacagcaagcagtagggcctggctgcaggacagggtgtgaagtgggggagcagtgatcaggagggccagagagatcagcagggatgtgatcttgagaagctgtgtgtgccatgatctggccctattaatccagaagggtctgatggaagcctctgtgattctcttccatggttaaacattttaattgtattatacctcggatattcctaaatatttaaaacactggcatggttgaactagacaacctttaagtagtttgttccaaccatgagatttagatttcatgatttaggttttatgatcttaaactgaaacctgttagttttctaccactagtgagatcatggcctctgcttttctcctgggaagtccctcttataatcactctcttcccatgattaaagggctactctgccttcatgttgctacccgctcccctggaaatggagaatcaagcaaggatgcggttttccttccattactacatccatacaagagtaaatcaagaataaaagtccagttaatgaaaagatcactggtcttaatatacttagcaaaattttaaaggcaattaaaagtatatacatagacaatgatcaaaattctaatgaaaagacccggctctcccctaaaagaagaaaaaatcatgtaatgtatatatgcattccataaaaacatacatggggaaaacttcagaagcctaaaaacaaaacatcagtaaaccaagccacacttagaaaaatgaaagctgatttttattttatcatcaacagccattctttagacatgaacatgcatacgtaatattctacgcacacatcacagcttttaacgttagttaataaaggttaaacacacaacatacatccttacaaaaaaagtcaaaatgcaaacttaaaactttaaacaaaagtattactaatttaaaaaaagtttgtgttgggtaccatttgtacaacacagttaatttaaacattttcattttggttgcacatgaaaaaggcggcagtagaaaataaagtcattgagggtttttaaatagcagaataggcagttttgccatgcaggagaagcaatattaaatattagtttcaaaaaaaatccacatttaaaaatatttagttcaagtcacagaatttttctcagtagagaccccaatgcaatgcataattagctgccttagatggcccgtttgaaaggatgatatcccttcagagtgtaactttactgattttggcacagaaaagaagtcttaagaacatgattaaaaaagagggaagaggaacagaggaaagaaataaaagcaagaataaatgagatagtaattgcaatcactaaaaaactgcattctcagtcattgcagaatactgtcttctgtctacagcaggtgcttattccagaattgttattgcagcatggatttaatttgcttggaggtagtctcatcattcaaatgttttgttgtgtacctgagagcatttagaagaccttccacactattaggaggttggtccttaagaactttgatacaacctttcatatcaattttggaagttttagcaaatgctcccactggatgtacgtggtcatagagtattatgacacccaccattaccctcaagcagaatgacactgtctcttcatttgtaaatctgcttctgtattccggtgtttccagcatgactctgcatacactagccattgtgcttaaacaatctgtggtattttctattggtaaatttttattctctgatacaaattttgttgtggcatcactcaaggttttcagcattggagttgcctcagcataaaacaaagacattcgatttgccaattcattatttacttcattttctccttctgccggtacattgttaatcctcatacgactcaatgttcttctataatagctgaaatcattctgtatggcaggatttgtcatcttgagttcatcaaaccggagtgtgaaatgaagaatttctgcaaactgtttagcaagagcctgctctcgctctagatgctgggtgggagaatatggggtacttgttaaggctcccagaagacctcttaatgctgcttctctcgtatttcgtggccagctcctctgtatgactgcaagtcctccaagatgccttctgcatcttttaatactacattcacctgattataaatttccttctcagactctgtaggctgggcattttcaaaatcaaggaaaaaatttggcccctgctcaaggtctgtgcatgtcaaaactttaagaagattccccatgttaaggtaccttcagccagtgctggtgattctgtccttgtccttctatcaactgggtaaccttgaatgagttaatcaaattccaggcctcagtttcttctcctggcggcccgggcgggcgaggggagcgcggcgcgggagcgcaggagcctcggagcctccggtgccgccgccgccgccgtttccgggttggcggggctcacgtcaccgccacaggtttgcgagctgcccccgccgcggcggcagcagcagcagcagcagcagcccgggcgagtgccaggcgagaaataact

SEQ ID NO: 18523 - RNA, 3092 nt, Homo sapiens
  source 1..3092: mol_type = other RNA
tgagctgctgtaccaaaataccacaaactgcatggcttaaaacaacagaaatttattccctcacaatcctggaggccagatgtctgaaatcaagatattggtagggttggttccttctcgagactctgagggagaatctgtgacatgcctgttttcctagcttctagtgacttcctccaattcttagggttctttggctcatagatgcattgctctaatctctgcctccatcttcccatggccttcagctctgtgtgtctatttccccttcttttctaagagctagtcattgaatttagggcccaccctactacaggttgatctcatttccaggtccttgatttcatctgcaaaaactttttccaaataatgtcacacgtggagattcccagtgaatgtatctcctgggggccactattcagcctattacactattcttagaagatgcctagaaggatatggccaatgttatccagaaggcttcatgaaggaggtaatagaagctaacccttcaaagatgaaagttggcgttcattagagggtcacaaggggaggaagggaatgtcaggttcagggaccagccagaccagagctaaggaagtgacatcacatggaacaatttgtgaacagcaagcagtagggcctggctgcaggacagggtgtgaagtgggggagcagtgatcaggagggccagagagatcagcagggatgtgatcttgagaagctgtgtgtgccatgatctggccctattaatccagaagggtctgatggaagcctctgtgattctcttccatggttaaacattttaattgtattatacctcggatattcctaaatatttaaaacactggcatggttgaactagacaacctttaagtagtttgttccaaccatgagatttagatttcatgatttaggttttatgatcttaaactgaaacctgttagttttctaccactagtgagatcatggcctctgcttttctcctgggaagtccctcttataatcactctcttcccatgattaaagggctactctgccttcatgttgctacccgctcccctggaaatggagaatcaagcaaggatgcggttttccttccattactacatccatacaagagtaaatcaagaataaaagtccagttaatgaaaagatcactggtcttaatatacttagcaaaattttaaaggcaattaaaagtatatacatagacaatgatcaaaattctaatgaaaagacccggctctcccctaaaagaagaaaaaatcatgtaatgtatatatgcattccataaaaacatacatggggaaaacttcagaagcctaaaaacaaaacatcagtaaaccaagccacacttagaaaaatgaaagctgatttttattttatcatcaacagccattctttagacatgaacatgcatacgtaatattctacgcacacatcacagcttttaacgttagttaataaaggttaaacacacaacatacatccttacaaaaaaagtcaaaatgcaaacttaaaactttaaacaaaagtattactaatttaaaaaaagtttgtgttgggtaccatttgtacaacacagttaatttaaacattttcattttggttgcacatgaaaaaggcggcagtagaaaataaagtcattgagggtttttaaatagcagaataggcagttttgccatgcaggagaagcaatattaaatattagtttcaaaaaaaatccacatttaaaaatatttagttcaagtcacagaatttttctcagtagagaccccaatgcaatgcataattagctgccttagatggcccgtttgaaaggatgatatcccttcagagtgtaactttactgattttggcacagaaaagaagtcttaagaacatgattaaaaaagagggaagaggaacagaggaaagaaataaaagcaagaataaatgagatagtaattgcaatcactaaaaaactgcattctcagtcattgcagaatactgtcttctgtctacagcaggtgcttattccagaattgttattgcagcatggatttaatttgcttggaggtagtctcatcattcaaatgttttgttgtgtacctgagagcatttagaagaccttccacactattaggaggttggtccttaagaactttgatacaacctttcatatcaattttggaagttttagcaaatgctcccactggatgtacgtggtcatagagtattatgacacccaccattaccctcaagcagaatgacactgtctcttcatttgtaaatctgcttctgtattccggtgtttccagcatgactctgcatacactagccattgtgcttaaacaatctgtggtattttctattggtaaatttttattctctgatacaaattttgttgtggcatcactcaaggttttcagcattggagttgcctcagcataaaacaaagacattcgatttgccaattcattatttacttcattttctccttctgccggtacattgttaatcctcatacgactcaatgttcttctataatagctgaaatcattctgtatggcaggatttgtcatcttgagttcatcaaaccggagtgtgaaatgaagaatttctgcaaactgtttagcaagagcctgctctcgctctagatgctgggtgggagaatatggggtacttgttaaggctcccagaagacctcttaatgctgcttctctcgtatttcgtggccagctcctctgtatgactgcaagtcctccaagatgccttctgcatcttttaatactacattcacctgattataaatttccttctcagactctgtaggctgggcattttcaaaatcaaggaaaaaatttggcccctgctcaaggtctgtgcatgtcaaaactttaagaagattccccatgttaaggtaccttcagccagtgctggtgattctgtccttgtccttctatcaactgggtaaccttgaatgagttaatcaaattccaggcctcagtttcttctccttcgagaagccgagccgccggcgctcgcacaaaaggaggacgctcgcctcgcgacgcgcctccccccgcgcccagtccccgccgcatcgc

SEQ ID NO: 18524 - RNA, 3279 nt, Homo sapiens
  source 1..3279: mol_type = other RNA
tgagctgctgtaccaaaataccacaaactgcatggcttaaaacaacagaaatttattccctcacaatcctggaggccagatgtctgaaatcaagatattggtagggttggttccttctcgagactctgagggagaatctgtgacatgcctgttttcctagcttctagtgacttcctccaattcttagggttctttggctcatagatgcattgctctaatctctgcctccatcttcccatggccttcagctctgtgtgtctatttccccttcttttctaagagctagtcattgaatttagggcccaccctactacaggttgatctcatttccaggtccttgatttcatctgcaaaaactttttccaaataatgtcacacgtggagattcccagtgaatgtatctcctgggggccactattcagcctattacactattcttagaagatgcctagaaggatatggccaatgttatccagaaggcttcatgaaggaggtaatagaagctaacccttcaaagatgaaagttggcgttcattagagggtcacaaggggaggaagggaatgtcaggttcagggaccagccagaccagagctaaggaagtgacatcacatggaacaatttgtgaacagcaagcagtagggcctggctgcaggacagggtgtgaagtgggggagcagtgatcaggagggccagagagatcagcagggatgtgatcttgagaagctgtgtgtgccatgatctggccctattaatccagaagggtctgatggaagcctctgtgattctcttccatggttaaacattttaattgtattatacctcggatattcctaaatatttaaaacactggcatggttgaactagacaacctttaagtagtttgttccaaccatgagatttagatttcatgatttaggttttatgatcttaaactgaaacctgttagttttctaccactagtgagatcatggcctctgcttttctcctgggaagtccctcttataatcactctcttcccatgattaaagggctactctgccttcatgttgctacccgctcccctggaaatggagaatcaagcaaggatgcggttttccttccattactacatccatacaagagtaaatcaagaataaaagtccagttaatgaaaagatcactggtcttaatatacttagcaaaattttaaaggcaattaaaagtatatacatagacaatgatcaaaattctaatgaaaagacccggctctcccctaaaagaagaaaaaatcatgtaatgtatatatgcattccataaaaacatacatggggaaaacttcagaagcctaaaaacaaaacatcagtaaaccaagccacacttagaaaaatgaaagctgatttttattttatcatcaacagccattctttagacatgaacatgcatacgtaatattctacgcacacatcacagcttttaacgttagttaataaaggttaaacacacaacatacatccttacaaaaaaagtcaaaatgcaaacttaaaactttaaacaaaagtattactaatttaaaaaaagtttgtgttgggtaccatttgtacaacacagttaatttaaacattttcattttggttgcacatgaaaaaggcggcagtagaaaataaagtcattgagggtttttaaatagcagaataggcagttttgccatgcaggagaagcaatattaaatattagtttcaaaaaaaatccacatttaaaaatatttagttcaagtcacagaatttttctcagtagagaccccaatgcaatgcataattagctgccttagatggcccgtttgaaaggatgatatcccttcagagtgtaactttactgattttggcacagaaaagaagtcttaagaacatgattaaaaaagagggaagaggaacagaggaaagaaataaaagcaagaataaatgagatagtaattgcaatcactaaaaaactgcattctcagtcattgcagaatactgtcttctgtctacagcaggtgcttattccagaattgttattgcagcatggatttaatttgcttggaggtagtctcatcattcaaatgttttgttgtgtacctgagagcatttagaagaccttccacactattaggaggttggtccttaagaactttgatacaacctttcatatcaattttggaagttttagcaaatgctcccactggatgtacgtggtcatagagtattatgacacccaccattaccctcaagcagaatgacactgtctcttcatttgtaaatctgcttctgtattccggtgtttccagcatgactctgcatacactagccattgtgcttaaacaatctgtggtattttctattggtaaatttttattctctgatacaaattttgttgtggcatcactcaaggttttcagcattggagttgcctcagcataaaacaaagacattcgatttgccaattcattatttacttcattttctccttctgccggtacattgttaatcctcatacgactcaatgttcttctataatagctgaaatcattctgtatggcaggatttgtcatcttgagttcatcaaaccggagtgtgaaatgaagaatttctgcaaactgtttagcaagagcctgctctcgctctagatgctgggtgggagaatatggggtacttgttaaggctcccagaagacctcttaatgctgcttctctcgtatttcgtggccagctcctctgtatgactgcaagtcctccaagatgccttctgcatcttttaatactacattcacctgattataaatttccttctcagactctgtaggctgggcattttcaaaatcaaggaaaaaatttggcccctgctcaaggtctgtgcatgtcaaaactttaagaagattccccatgttaaggtaccttcagccagtgctggtgattctgtccttgtccttctatccttggattggcgttccctctttcctagttcacttgttccagtccttcaacttctgtttcttgctaacaggtgtgcaaatgaattaccaactgggtaaccttgaatgagttaatcaaattccaggcctcagtttcttctcctggcggcccgggcgggcgaggggagcgcggcgcgggagcgcaggagcctcggagcctccggtgccgccgccgccgccgtttccgggttggcggggctcacgtcaccgccacaggtttgcgagctgcccccgccgcggcggcagcagcagcagcagcagcagcccgggcgagtgccaggcgagaaataact

SEQ ID NO: 18525 - RNA, 3239 nt, Homo sapiens
  source 1..3239: mol_type = other RNA
tgagctgctgtaccaaaataccacaaactgcatggcttaaaacaacagaaatttattccctcacaatcctggaggccagatgtctgaaatcaagatattggtagggttggttccttctcgagactctgagggagaatctgtgacatgcctgttttcctagcttctagtgacttcctccaattcttagggttctttggctcatagatgcattgctctaatctctgcctccatcttcccatggccttcagctctgtgtgtctatttccccttcttttctaagagctagtcattgaatttagggcccaccctactacaggttgatctcatttccaggtccttgatttcatctgcaaaaactttttccaaataatgtcacacgtggagattcccagtgaatgtatctcctgggggccactattcagcctattacactattcttagaagatgcctagaaggatatggccaatgttatccagaaggcttcatgaaggaggtaatagaagctaacccttcaaagatgaaagttggcgttcattagagggtcacaaggggaggaagggaatgtcaggttcagggaccagccagaccagagctaaggaagtgacatcacatggaacaatttgtgaacagcaagcagtagggcctggctgcaggacagggtgtgaagtgggggagcagtgatcaggagggccagagagatcagcagggatgtgatcttgagaagctgtgtgtgccatgatctggccctattaatccagaagggtctgatggaagcctctgtgattctcttccatggttaaacattttaattgtattatacctcggatattcctaaatatttaaaacactggcatggttgaactagacaacctttaagtagtttgttccaaccatgagatttagatttcatgatttaggttttatgatcttaaactgaaacctgttagttttctaccactagtgagatcatggcctctgcttttctcctgggaagtccctcttataatcactctcttcccatgattaaagggctactctgccttcatgttgctacccgctcccctggaaatggagaatcaagcaaggatgcggttttccttccattactacatccatacaagagtaaatcaagaataaaagtccagttaatgaaaagatcactggtcttaatatacttagcaaaattttaaaggcaattaaaagtatatacatagacaatgatcaaaattctaatgaaaagacccggctctcccctaaaagaagaaaaaatcatgtaatgtatatatgcattccataaaaacatacatggggaaaacttcagaagcctaaaaacaaaacatcagtaaaccaagccacacttagaaaaatgaaagctgatttttattttatcatcaacagccattctttagacatgaacatgcatacgtaatattctacgcacacatcacagcttttaacgttagttaataaaggttaaacacacaacatacatccttacaaaaaaagtcaaaatgcaaacttaaaactttaaacaaaagtattactaatttaaaaaaagtttgtgttgggtaccatttgtacaacacagttaatttaaacattttcattttggttgcacatgaaaaaggcggcagtagaaaataaagtcattgagggtttttaaatagcagaataggcagttttgccatgcaggagaagcaatattaaatattagtttcaaaaaaaatccacatttaaaaatatttagttcaagtcacagaatttttctcagtagagaccccaatgcaatgcataattagctgccttagatggcccgtttgaaaggatgatatcccttcagagtgtaactttactgattttggcacagaaaagaagtcttaagaacatgattaaaaaagagggaagaggaacagaggaaagaaataaaagcaagaataaatgagatagtaattgcaatcactaaaaaactgcattctcagtcattgcagaatactgtcttctgtctacagcaggtgcttattccagaattgttattgcagcatggatttaatttgcttggaggtagtctcatcattcaaatgttttgttgtgtacctgagagcatttagaagaccttccacactattaggaggttggtccttaagaactttgatacaacctttcatatcaattttggaagttttagcaaatgctcccactggatgtacgtggtcatagagtattatgacacccaccattaccctcaagcagaatgacactgtctcttcatttgtaaatctgcttctgtattccggtgtttccagcatgactctgcatacactagccattgtgcttaaacaatctgtggtattttctattggtaaatttttattctctgatacaaattttgttgtggcatcactcaaggttttcagcattggagttgcctcagcataaaacaaagacattcgatttgccaattcattatttacttcattttctccttctgccggtacattgttaatcctcatacgactcaatgttcttctataatagctgaaatcattctgtatggcaggatttgtcatcttgagttcatcaaaccggagtgtgaaatgaagaatttctgcaaactgtttagcaagagcctgctctcgctctagatgctgggtgggagaatatggggtacttgttaaggctcccagaagacctcttaatgctgcttctctcgtatttcgtggccagctcctctgtatgactgcaagtcctccaagatgccttctgcatcttttaatactacattcacctgattataaatttccttctcagactctgtaggctgggcattttcaaaatcaaggaaaaaatttggcccctgctcaaggtctgtgcatgtcaaaactttaagaagattccccatgttaaggtaccttcagccagtgctggtgattctgtccttgtccttctatccttggattggcgttccctctttcctagttcacttgttccagtccttcaacttctgtttcttgctaacaggtgtgcaaatgaattaccctccgctcgagcctccaggcgctctcagtcccgctcctgcgccctcctggagccgcagaggcggctcctcagcggcgctagggggagccccgggtccggagcgggggagcggcggcagccggaccgggagcccctcaacacctgcccctgtggcagagccgcgacaagccaggcggcagctccgagcggggagggcaagtgac

SEQ ID NO: 18526 - RNA, 3239 nt, Homo sapiens
  source 1..3239: mol_type = other RNA
tgagctgctgtaccaaaataccacaaactgcatggcttaaaacaacagaaatttattccctcacaatcctggaggccagatgtctgaaatcaagatattggtagggttggttccttctcgagactctgagggagaatctgtgacatgcctgttttcctagcttctagtgacttcctccaattcttagggttctttggctcatagatgcattgctctaatctctgcctccatcttcccatggccttcagctctgtgtgtctatttccccttcttttctaagagctagtcattgaatttagggcccaccctactacaggttgatctcatttccaggtccttgatttcatctgcaaaaactttttccaaataatgtcacacgtggagattcccagtgaatgtatctcctgggggccactattcagcctattacactattcttagaagatgcctagaaggatatggccaatgttatccagaaggcttcatgaaggaggtaatagaagctaacccttcaaagatgaaagttggcgttcattagagggtcacaaggggaggaagggaatgtcaggttcagggaccagccagaccagagctaaggaagtgacatcacatggaacaatttgtgaacagcaagcagtagggcctggctgcaggacagggtgtgaagtgggggagcagtgatcaggagggccagagagatcagcagggatgtgatcttgagaagctgtgtgtgccatgatctggccctattaatccagaagggtctgatggaagcctctgtgattctcttccatggttaaacattttaattgtattatacctcggatattcctaaatatttaaaacactggcatggttgaactagacaacctttaagtagtttgttccaaccatgagatttagatttcatgatttaggttttatgatcttaaactgaaacctgttagttttctaccactagtgagatcatggcctctgcttttctcctgggaagtccctcttataatcactctcttcccatgattaaagggctactctgccttcatgttgctacccgctcccctggaaatggagaatcaagcaaggatgcggttttccttccattactacatccatacaagagtaaatcaagaataaaagtccagttaatgaaaagatcactggtcttaatatacttagcaaaattttaaaggcaattaaaagtatatacatagacaatgatcaaaattctaatgaaaagacccggctctcccctaaaagaagaaaaaatcatgtaatgtatatatgcattccataaaaacatacatggggaaaacttcagaagcctaaaaacaaaacatcagtaaaccaagccacacttagaaaaatgaaagctgatttttattttatcatcaacagccattctttagacatgaacatgcatacgtaatattctacgcacacatcacagcttttaacgttagttaataaaggttaaacacacaacatacatccttacaaaaaaagtcaaaatgcaaacttaaaactttaaacaaaagtattactaatttaaaaaaagtttgtgttgggtaccatttgtacaacacagttaatttaaacattttcattttggttgcacatgaaaaaggcggcagtagaaaataaagtcattgagggtttttaaatagcagaataggcagttttgccatgcaggagaagcaatattaaatattagtttcaaaaaaaatccacatttaaaaatatttagttcaagtcacagaatttttctcagtagagaccccaatgcaatgcataattagctgccttagatggcccgtttgaaaggatgatatcccttcagagtgtaactttactgattttggcacagaaaagaagtcttaagaacatgattaaaaaagagggaagaggaacagaggaaagaaataaaagcaagaataaatgagatagtaattgcaatcactaaaaaactgcattctcagtcattgcagaatactgtcttctgtctacagcaggtgcttattccagaattgttattgcagcatggatttaatttgcttggaggtagtctcatcattcaaatgttttgttgtgtacctgagagcatttagaagaccttccacactattaggaggttggtccttaagaactttgatacaacctttcatatcaattttggaagttttagcaaatgctcccactggatgtacgtggtcatagagtattatgacacccaccattaccctcaagcagaatgacactgtctcttcatttgtaaatctgcttctgtattccggtgtttccagcatgactctgcatacactagccattgtgcttaaacaatctgtggtattttctattggtaaatttttattctctgatacaaattttgttgtggcatcactcaaggttttcagcattggagttgcctcagcataaaacaaagacattcgatttgccaattcattatttacttcattttctccttctgccggtacattgttaatcctcatacgactcaatgttcttctataatagctgaaatcattctgtatggcaggatttgtcatcttgagttcatcaaaccggagtgtgaaatgaagaatttctgcaaactgtttagcaagagcctgctctcgctctagatgctgggtgggagaatatggggtacttgttaaggctcccagaagacctcttaatgctgcttctctcgtatttcgtggccagctcctctgtatgactgcaagtcctccaagatgccttctgcatcttttaatactacattcacctgattataaatttccttctcagactctgtaggctgggcattttcaaagtccaagaaaaaatgtgctgcattgtggtctatgtccctggttagcaccttaatgagattacccatgccagcaaaccttcagccagtgctggtgattctgtccttgtccttctatccttggattggcgttccctctttcctagttcacttgttccagtccttcaacttctgtttcttgctaacaggtgtgcaaatgaattaccctccgctcgagcctccaggcgctctcagtcccgctcctgcgccctcctggagccgcagaggcggctcctcagcggcgctagggggagccccgggtccggagcgggggagcggcggcagccggaccgggagcccctcaacacctgcccctgtggcagagccgcgacaagccaggcggcagctccgagcggggagggcaagtgac

SEQ ID NO: 18527 - RNA, 728 nt, Homo sapiens
  source 1..728: mol_type = other RNA
tgagctgctgtaccaaaatgacctgggaatccccgagccaggcgacgtgcagggtcgctcctgcaatgagcgcacacacacctgtggtgccgctctgcagccgctctcgcttggctttcctgagaaacatctggtcggtgcgccggaaggcttctctgagggctccctcagggtctgtgggcagctctggctggcgggcagcgttggtgtgcacgtggacagcggcgtacctcgcagcatccacgcctccgtgaccatcaaacacagcaaagtaggcgcggttcacagggtcagacaagccgaagagctggttgaaggaagggagggacacgtgccggtcctccatcttgcggcgagtgttccggatggcgtggatggagaccagccactgccgctgtgaggcccgggcagccaatggcacctgcttctgccactggccggcgacttcccaaaggcggttaaagaaactctgtgccaggctttgggcatccagcaaggtcacaggggccttttcctcctcgtcatcgtcctcctcctcttcttcttcctccctgggcaacttcctgaattcggaaaggtctgtctgtagcagctgtgaaactgcttcgtgggccagagcagcagcaagtggtggcggggccttcccctggtctccgcgggcctcagctgtctcctcgcggctccgtgtcccgcaagctgctgccggccggccccgcccacttcccgtc

SEQ ID NO: 18528 - RNA, 967 nt, Homo sapiens
  source 1..967: mol_type = other RNA
tgagctgctgtaccaaaatgacctgggaatccccgagccaggcgacgtgcagggtcgctcctgcaatgagcgcacacacacctgtggtgccgctctgcagccgctctcgcttggctttcctgagaaacatctggtcggtgcgccggaaggcttctctgagggctccctcagggtctgtgggcagctctggctggcgggcagcgttggtgtgcacgtggacagcggcgtacctcgcagcatccacgcctccgtgaccatcaaacacagcaaagtaggcgcggttcacagggtcagacaagccgaagagctggttgaaggaagggagggacacgtgccggtcctccatcttgcggcgagtgttccggatggcgtggatggagaccagccactgccgctgtgaggcccgggcagccaatggcacctgcttctgccactggccggcgacttcccaaaggcggttaaagaaactctgtgccaggctttgggcatccagcaaggtcacaggggccttttcctcctcgtcatcgtcctcctcctcttcttcttcctccctgggcaacttcctgaattcggaaaggtctgtctgtagcagctgtgaaactgcttcgtgggccagagcagcagcaagtggtggcggggccttcctgctgcccagaaagcccatggccagctcagccagctcgccctccacctcctcctggctgagcaccgtccctggggccttccatggcagagggtcctctgggttcagcagggctgggaagtcttgcaggagcgtgtccaggaagcctggggtctcctcagctccactggccattgggctgctcttctgtggggctccagaggacatgcccaaagcatcccgggggcctgcagctaggccagggcaagagggtctccaggcttcaccccctggtctccgcgggcctcagctgtctcctcgcggctccgtgtcccgcaagctgct

SEQ ID NO: 18529 - RNA, 31 nt, Homo sapiens
  source 1..31: mol_type = other RNA
tgaggagatcgtcgaggttggcctgcttccc

SEQ ID NO: 18530 - RNA, 2585 nt, Homo sapiens
  source 1..2585: mol_type = other RNA
tgaggatatggcagggaaggggaggttctgtgatggatgctttccccagaagcctgatacgcagtggccagggagactgagtcccgggagagggtttggggtgggagaggtctgagcatgaggggcagggcacactctggttcagggagatgtaggacaaaggactctggccttgggactgatctgggctggtttccttacattcctctcaggcccttccccctgtatgctaaggggggatggtacctggacttcaagaccaaaagcccttctctgaccgcactgctgagtgcagcaggcagctccacccacagtctctgggcagccccaggctgtcccctccccactctgattctaggacaaagaccttggacctcagctggatgctggggatcaggagaggaggaatggtaggtgtggaaacaaggggcaggattcggggtgagcagagctgggggctgcagaccttgctcaggacagtcctaatgcctgcaagctcctaacgccctccccacattcccttttctacatggggagctcctacactgtgtcccctcacctatcgctgatccccagcatccagctggagggccttccaggaactgtcccttcccttaggaggtctctggagcacagtaacaggggcagggtttactaccttggggcctctttccacaccaggggctccctgaccctggggactgctcctagagctgggccaagcctcaggggcagcctccaggagtgagtgggatctcctatcaaggaggactttgtgccaaggccaaggccaggcttgggaggggggtccctagacagagggtaggacctctgaattatttcttgcttagccctggatgtgctatgtaacccaccctggacctctgtctcctcatctttctgcccaagagccccaggggtcagcactgaccactctgacacaggccccgtccaagccacgctgaggacagaccgaatgataccatgattggggctggatgttcacttctctttccaaaaaaatatgaaacacacagtctaggtatggcaggggacagagcctggctggggactggacattacacacccagggggcccttggcggaggcgggcaatttaacaactggtctgaaagtcaaaagagagagagctggttagtggagtgagctgtggggtcgggggcaggggctgtgcattcaggcccggacatgggtactggccagcgtggccagaccttggccctcacagcagccctgcctggggcccattcccgggggcaggggcgccatggtccgacctcaccatctgtgtaggtggcccccagccctgggcgcactggaagaacctgagacctaaactcagaccctccctgtccttgtgtgaacgttcagcatcccggcactgcccttgtggggttgctgtgaggagcccatgggactggggagggtgaaggtttctgctcaccccaaggacctgggtactaaggtacgtcttggccactgctctatctctagggcccagcacgtagcagacacccaagcagctcttcagtgagtaaacagccgggctggtgcctgagggcctgtctccagggatgcatgctggtgcccaccaggctgtgcagacaagaccgtgcctggacctgcatctgtgtgtatgcctgggggctgggtcctgcctctggtgtctctctgaggatctgggtctcagattgcagggtgggtgcttgtgttgaggacaagctgctcagagcacctatgcccatcctatgccccagtggccctgcccagggtgctgcgaggctggctggatgctgggcaagggggccactgggtggggggctggccagggcaggcggagctcagacgtactctcgggcagcagcagagggtccaggccgatagggctgtgggctgctgttgggtctctctggctccgggcatgtgcagcagaggaaggagccgcccagcacggccaggccagctgaggcccagcccacgaacagggctgggccaaattcatacctgccaggatgaagagggctcccccggcgatggcaacacggcccttggcaatggggttgctgtctcccacccgcgtacacttcatgccaactacgctgaggaccatggccacgaagcccaggagcacggccaccaccatcagggcccgcgctgattggatgtgaccgtccagggcgagcagcgagtcgtagagcttgcactgcacttgcccagtgctctgggaggcgcaggacatccagagcccttcatagaggcccacggcagtgatgatggcgtcgcctgcgtaggaagactgcttccactgtggcagggctgtgctagcaatgatgcccacccagccacccagggccaagaagtagcccaggagctggaggcctgagttggccatggcccaggagagaggaccgagggtcccaggactcagagctgggccagggtgccagcaggggctttggtcatggccaggtgggaggagcagctgggcagggggagcagcgagaaggagggtcagaggcagagaaggagaggtggtgcggcggcagcggctggagcaaaggcagt

SEQ ID NO: 18531 - RNA, 2670 nt, Homo sapiens
  source 1..2670: mol_type = other RNA
tgaggatatggcagggaaggggaggttctgtgatggatgctttccccagaagcctgatacgcagtggccagggagactgagtcccgggagagggtttggggtgggagaggtctgagcatgaggggcagggcacactctggttcagggagatgtaggacaaaggactctggccttgggactgatctgggctggtttccttacattcctctcaggcccttccccctgtatgctaaggggggatggtacctggacttcaagaccaaaagcccttctctgaccgcactgctgagtgcagcaggcagctccacccacagtctctgggcagccccaggctgtcccctccccactctgattctaggacaaagaccttggacctcagctggatgctggggatcaggagaggaggaatggtaggtgtggaaacaaggggcaggattcggggtgagcagagctgggggctgcagaccttgctcaggacagtcctaatgcctgcaagctcctaacgccctccccacattcccttttctacatggggagctcctacactgtgtcccctcacctatcgctgatccccagcatccagctggagggccttccaggaactgtcccttcccttaggaggtctctggagcacagtaacaggggcagggtttactaccttggggcctctttccacaccaggggctccctgaccctggggactgctcctagagctgggccaagcctcaggggcagcctccaggagtgagtgggatctcctatcaaggaggactttgtgccaaggccaaggccaggcttgggaggggggtccctagacagagggtaggacctctgaattatttcttgcttagccctggatgtgctatgtaacccaccctggacctctgtctcctcatctttctgcccaagagccccaggggtcagcactgaccactctgacacaggccccgtccaagccacgctgaggacagaccgaatgataccatgattggggctggatgttcacttctctttccaaaaaaatatgaaacacacagtctaggtatggcaggggacagagcctggctggggactggacattacacacccagggggcccttggcggaggcgggcaatttaacaactggtctgaaagtcaaaagagagagagctggttagtggagtgagctgtggggtcgggggcaggggctgtgcattcaggcccggacatgggtactggccagcgtggccagaccttggccctcacagcagccctgcctggggcccattcccgggggcaggggcgccatggtccgacctcaccatctgtgtaggtggcccccagccctgggcgcactggaagaacctgagacctaaactcagaccctccctgtccttgtgtgaacgttcagcatcccggcactgcccttgtggggttgctgtgaggagcccatgggactggggagggtgaaggtttctgctcaccccaaggacctgggtactaaggtacgtcttggccactgctctatctctagggcccagcacgtagcagacacccaagcagctcttcagtgagtaaacagccgggctggtgcctgagggcctgtctccagggatgcatgctggtgcccaccaggctgtgcagacaagaccgtgcctggacctgcatctgtgtgtatgcctgggggctgggtcctgcctctggtgtctctctgaggatctgggtctcagattgcagggtgggtgcttgtgttgaggacaagctgctcagagcacctatgcccatcctatgccccagtggccctgcccagggtgctgcgaggctggctggatgctgggcaagggggccactgggtggggggctggccagggcaggcggagctcagacgtactctcgggcagcagcagagggtccaggccgatagggctgtgggctgctgttgggtctctctggctccgggcatgtgcagcagaggaaggagccgcccagcacggccaggccagctgaggcccagcccacgaacagggctgggccaaattcatacctggcattgacaggtgtgcttgggttgaagaactcctgggtcaccagggtggcataccacgagacagcagtcaaagtgcagaggcctgccaggatgaagagggctcccccggcgatggcaacacggcccttggcaatggggttgctgtctcccacccgcgtacacttcatgccaactacgctgaggaccatggccacgaagcccaggagcacggccaccaccatcagggcccgcgctgattggatgtgaccgtccagggcgagcagcgagtcgtagagcttgcactgcacttgcccagtgctctgggaggcgcaggacatccagagcccttcatagaggcccacggcagtgatgatggcgtcgcctgcgtaggaagactgcttccactgtggcagggctgtgctagcaatgatgcccacccagccacccagggccaagaagtagcccaggagctggaggcctgagttggccatggcccaggagagaggaccgagggtcccaggactcagagctgggccagggtgccagcaggggctttggtcatggccaggtgggaggagcagctgggcagggggagcagcgagaaggagggtcagaggcagagaaggagaggtggtgcggcggcagcggctggagcaaaggcagt

SEQ ID NO: 18532 - RNA, 1927 nt, Homo sapiens
  source 1..1927: mol_type = other RNA
tgaggatatggcagggaaggggaggttctgtgatggatgctttccccagaagcctgatacgcagtggccagggagactgagtcccgggagagggtttggggtgggagaggtctgagcatgaggggcagggcacactctggttcagggagatgtaggacaaaggactctggccttgggactgatctgggctggtttccttacattcctctcaggcccttccccctgtatgctaaggggggatggtacctggacttcaagaccaaaagcccttctctgaccgcactgctgagtgcagcaggcagctccacccacagtctctgggcagccccaggctgtcccctccccactctgattctaggacaaagaccttggacctcagctggatgctggggatcaggagaggaggaatggtaggtgtggaaacaaggggcaggattcggggtgagcagagctgggggctgcagaccttgctcaggacagtcctaatgcctgcaagctcctaacgccctccccacattcccttttctacatggggagctcctacactgtgtcccctcacctatcgctgatccccagcatccagctggagggccttccaggaactgtcccttcccttaggaggtctctggagcacagtaacaggggcagggtttactaccttggggcctctttccacaccaggggctccctgaccctggggactgctcctagagctgggccaagcctcaggggcagcctccaggagtgagtgggatctcctatcaaggaggactttgtgccaaggccaaggccaggcttgggaggggggtccctagacagagggtaggacctctgaattatttcttgcttagccctggatgtgctatgtaacccaccctggacctctgtctcctcatctttctgcccaagagccccaggggtcagcactgaccactctgacacaggccccgtccaagccacgctgaggacagaccgaatgataccatgattggggctggatgttcacttctctttccaaaaaaatatgaaacacacagtctaggtatggcaggggacagagcctggctggggactggacattacacacccagggggcccttggcggaggcgggcaatttaacaactggttctcgggcagcagcagagggtccaggccgatagggctgtgggctgctgttgggtctctctggctccgggcatgtgcagcagaggaaggagccgcccagcacggccaggccagctgaggcccagcccacgaacagggctgggccaaattcatacctggcattgacaggtgtgcttgggttgaagaactcctgggtcaccagggtggcataccacgagacagcagtcaaagtgcagaggcctgccaggatgaagagggctcccccggcgatggcaacacggcccttggcaatggggttgctgtctcccacccgcgtacacttcatgccaactacgctgaggaccatggccacgaagcccaggagcacggccaccaccatcagggcccgcgctgattggatgtgaccgtccagggcgagcagcgagtcgtagagcttgcactgcacttgcccagtgctctgggaggcgcaggacatccagagcccttcatagaggcccacggcagtgatgatggcgtcgcctgcgtaggaagactgcttccactgtggcagggctgtgctagcaatgatgcccacccagccacccagggccaagaagtagcccaggagctggaggcctgagttggccatggcccaggagagaggaccgagggtcccaggactcagagctgggccagggtgccagcaggggctttggtcatggccaggtgggaggagcagctgggcagggggagcagcgagaaggagggtcagaggcagagaaggagaggtggtgcggcggcagcggctggagcaaaggcagt

SEQ ID NO: 18533 - RNA, 3155 nt, Homo sapiens
  source 1..3155: mol_type = other RNA
tgaggatatggcagggaaggggatagctacaggtgagcctgccttacggcatggcggacgcactcattcatcatgcgctgcacgcacggttctgcagcactcactccagcacacgactgtgctgccacgcacgtgttaggtgctacgggttcaacaatgataaggcactgtccctgccctcaaggagcttacggtctaggggggtgacattagactcccagcccacagagacacagctctggggagggatggggaagctcagttgctcggtgggtggggttagggcctcaccagctccctctggctgctcttagtggggaggtctgtgcttgtctggagtttgtctggaggccactgagtatgagacacctgcagtccctgtcttccttccccagcccccgaggaggagcacagttctcttcaggctcatcagtgccaggggactcttttcagtgactgataaaatggtcttcctcttcctctggtccataaggaaaaggtgtacttttctgaagcagcagaaaccagctgggagaaaatgaaaattagccttcagtctgcctaactcaagcctgccctcgggcttgtggtaaaaacttcatgtcgtaatccaggcgtgggagagagccgtggggtccactcagcctgggaatgtcccccgctggagggcctcgccctctgggtcaggtcagagcaggcatcgaggtgccctctccggtgccgccgccccaggccgagcctcccactccgggcccgccttcggtgcggacggagatcagtggttctgagcacactacacaatgctacggaggcctccagtgacacagtatttcctactcttacacatcggctgactggatggccagtaaaaagatgcagtggaggtgagctttccagttcatgggaagctccaagcagcctgcctgctgcaacacgactttggccacaggcgggagaggcagtacaaagctgtgtgatctggaggaagccacagtgtctgagatgggatctcatctgaaaccctggagccgtggcattgcttccttctatgtcaagataacgaaagcccgtggtatcagctggcttcattctattccattctattttggctgttgcagaaaaacattcttctgttccactgccttctgttcacagtctgtcagctcgaaacgtctcttcaacagaggggtccagcaggcccatgctggagtcacttaacatgttgagtccgtccaggctcaggggttcaatctgcagctcctcttccagtggaaatggagtgtccacgttcaggctgacctcaggcaggcctgccagcgcactgttgaggtctttgaacaggctggtgctggagtctggcaggatggtgttcgggagactcccgcagttggaatacgggcttggtctcaaatgaaaagagtcctgcagttctcgggaaccttgttgcaccagaggcacctgttgaggaaaggcagggcctggcctcatggactgctggtcaaaacccacatctgggaagaagttggtcaaagatgagccctgggccgggagaagctgaaagtctgactgtggcagtgaggaggctgcctggggctgctgggcaggggcctcaggggcgcggggctgctgcaggaggggctgggtgagctcctggggtgcagggtaagggggtggcggcgacacctgggcttgagcttctgtgggcagaaaggaaagttggcttcggtctgaggacaccatctgggaggtaggatatggggccagtgggctggttgaagacagctgtctgctgaaaccttgatgtgcttcagggccaggagaaagcgtgagagggctgacgggaggctgccgacgccgagacgggccgctcaggtttgtggtggaaagagatgggttgctaagggaaaacagacggagcgaagggtgaagagcagatgcgttgggaacagatgtctgtgggtggttatttaaggaagaggaaagcacagtcttattgagcgtggcttggatggaggggttactccgagaactctggagaccagaggagcttcttatacccaggtgggtcatagcagctgggatgttgttcacactattccccacactcatactgccaaagtggtggtcggtggtgtccagggaggctggcaggggtgtcgagtagtggaggttggttagatctggcaatgaccctccagtgttcaaggtccccaagaagggtgagaggcctaggttttgaccattatgtggaaaagcattgccacctccaacatcacaggatcgagggcgtcctgacagggactgaatctccttggtctcccacagttgttttggcagtggcttcggaacatttaacagattctcttctttcaatgggccagggaaagatgctacttccccatgtccattattctcaccatcacagaaacccatgtatggggcaggccaggccgactggccccctcctccataggggtcctggggcttggtactcagagcactcgtgtgaagagcagaatcagaattggtcctgttaagtgcagatgtcagcctgaacccaggatgcttttcgtctttccaaggaggctgctgccttggccaactctcatccagaggctgtgaggaataattggctccaaaagcactaccatcaaattgtcgccctggcttgtccccagaccttcggtggagggggtggaagcggttcctggatggcctctccaccagcccgtgatggcgggttccccgaacattatcagcttggtgaaatgacggctgaaactctgacgcactgctccgcagctggctcacatttggtaaggatcctccatggtactgtgtaaggcgcagttgctgaagcttctgaaattgaacccgcgacagggtgaggtcggtcatgagctgctcgaaggcccgcgtctcctcggcctgtctctgcgtgtgcagcgcgatcttctcactgaacttccgcgggttggcgctgcccgagcccggcgaggcggccatggcgcggactctgcgcgggcagaagcgggagacggcggccgtggggcctgtacctcggcccacccgtccgtccacaggccgccggggccgccgcccgaagccagtcgtccggcgcgacccggcagaggagccgccgcggccccggagcc

SEQ ID NO: 18534 - RNA, 3067 nt, Homo sapiens
  source 1..3067: mol_type = other RNA
tgaggatatggcagggaaggggatagctacaggtgagcctgccttacggcatggcggacgcactcattcatcatgcgctgcacgcacggttctgcagcactcactccagcacacgactgtgctgccacgcacgtgttaggtgctacgggttcaacaatgataaggcactgtccctgccctcaaggagcttacggtctaggggggtgacattagactcccagcccacagagacacagctctggggagggatggggaagctcagttgctcggtgggtggggttagggcctcaccagctccctctggctgctcttagtggggaggtctgtgcttgtctggagtttgtctggaggccactgagtatgagacacctgcagtccctgtcttccttccccagcccccgaggaggagcacagttctcttcaggctcatcagtgccaggggactcttttcagtgactgataaaatggtcttcctcttcctctggtccataaggaaaaggtgtacttttctgaagcagcagaaaccagctgggagaaaatgaaaattagccttcagtctgcctaactcaagcctgccctcgggcttgtggtaaaaacttcatgtcgtaatccaggcgtgggagagagccgtggggtccactcagcctgggaatgtcccccgctggagggcctcgccctctgggtcaggtcagagcaggcatcgaggtgccctctccggtgccgccgccccaggccgagcctcccactccgggcccgccttcggtgcggacggagatcagtggttctgagcacactacacaatgctacggaggcctccagtgacacagtatttcctactcttacacatcggctgactggatggccagtaaaaagatgcagtggaggtgagctttccagttcatgggaagctccaagcagcctgcctgctgcaacacgactttggccacaggcgggagaggcagtacaaagctgtgtgatctggaggaagccacagtgtctgagatgggatctcatctgaaaccctggagccgtggcattgcttccttctatgtcaagataacgaaagcccgtggtatcagctggcttcattctattccattctattttggctgttgcagaaaaacattcttctgttccactgccttctgttcacagtctgtcagctcgaaacgtctcttcaacagaggggtccagcaggcccatgctggagtcacttaacatgttgagtccgtccaggctcaggggttcaatctgcagctcctcttccagtggaaatggagtgtccacgttcaggctgacctcaggcaggcctgccagcgcactgttgaggtctttgaacaggctggtgctggagtcttctggcaggatggtgttcgggagactcccgcagttggaatacgggcttggtctcaaatgaaaagagtcctgcagttctcgggaaccttgttgcaccagaggcacctgttgaggaaaggcagggcctggcctcatggactgctggtcaaaacccacatctgggaagaagttggtcaaagatgagccctgggccgggagaagctgaaagtctgactgtggcagtgaggaggctgcctggggctgctgggcaggggcctcaggggcgcggggctgctgcaggaggggctgggtgagctcctggggtgcagggtaagggggtggcggcgacacctgggcttgagcttctgtgggcagaaaggaaagttggcttcggtctgaggacaccatctgggaggtaggatatggggccagtgggctggttgaagacagctgtctgctgaaaccttgatgtgcttcagggccaggagaaagcgtgagagggctgacgggaggctgccgacgccgagacgggccgctcaggtttgtggtggaaagagatgggttgctaagggaaaacagacggagcgaagggtgaagagcagatgcgttgggaacagatgtctgtgggtggttatttaaggaagaggaaagcacagtcttattgagcgtggcttggatggaggggttactccgagaactctggagaccagaggagcttcttatacccaggtgggtcatagcagctgggatgttgttcacactattccccacactcatactgccaaagtggtggtcggtggtgtccagggaggctggcaggggtgtcgagtagtggaggttggttagatctggcaatgaccctccagtgttcaaggtccccaagaagggtgagaggcctaggttttgaccattatgtggaaaagcattgccacctccaacatcacaggatcgagggcgtcctgacagggactgaatctccttggtctcccacagttgttttggcagtggcttcggaacatttaacagattctcttctttcaatgggccagggaaagatgctacttccccatgtccattattctcaccatcacagaaacccatgtatggggcaggccaggccgactggccccctcctccataggggtcctggggcttggtactcagagcactcgtgtgaagagcagaatcagaattggtcctgttaagtgcagatgtcagcctgaacccaggatgcttttcgtctttccaaggaggctgctgccttggccaactctcatccagaggctgtgaggaataattggctccaaaagcactaccatcaaattgtcgccctggcttgtccccagaccttcggtggagggggtggaagcggttcctggatggcctctccaccagcccgtgatggcgggttccccgaacattatcagcttggtgaaatgacggccgcgacagggtgaggtcggtcatgagctgctcgaaggcccgcgtctcctcggcctgtctctgcgtgtgcagcgcgatcttctcactgaacttccgcgggttggcgctgcccgagcccggcgaggcggccatggcgcggactctgcgcgggcagaagcgggagacggcggccgtggggcctgtacctcggcccacccgtccgtccacaggccgccggggccgccgcccgaagccagtcgtccggcgcgacccggcagaggagccgccgcggccccggagccagcgagcg

SEQ ID NO: 18535 - RNA, 3158 nt, Homo sapiens
  source 1..3158: mol_type = other RNA
tgaggatatggcagggaaggggatagctacaggtgagcctgccttacggcatggcggacgcactcattcatcatgcgctgcacgcacggttctgcagcactcactccagcacacgactgtgctgccacgcacgtgttaggtgctacgggttcaacaatgataaggcactgtccctgccctcaaggagcttacggtctaggggggtgacattagactcccagcccacagagacacagctctggggagggatggggaagctcagttgctcggtgggtggggttagggcctcaccagctccctctggctgctcttagtggggaggtctgtgcttgtctggagtttgtctggaggccactgagtatgagacacctgcagtccctgtcttccttccccagcccccgaggaggagcacagttctcttcaggctcatcagtgccaggggactcttttcagtgactgataaaatggtcttcctcttcctctggtccataaggaaaaggtgtacttttctgaagcagcagaaaccagctgggagaaaatgaaaattagccttcagtctgcctaactcaagcctgccctcgggcttgtggtaaaaacttcatgtcgtaatccaggcgtgggagagagccgtggggtccactcagcctgggaatgtcccccgctggagggcctcgccctctgggtcaggtcagagcaggcatcgaggtgccctctccggtgccgccgccccaggccgagcctcccactccgggcccgccttcggtgcggacggagatcagtggttctgagcacactacacaatgctacggaggcctccagtgacacagtatttcctactcttacacatcggctgactggatggccagtaaaaagatgcagtggaggtgagctttccagttcatgggaagctccaagcagcctgcctgctgcaacacgactttggccacaggcgggagaggcagtacaaagctgtgtgatctggaggaagccacagtgtctgagatgggatctcatctgaaaccctggagccgtggcattgcttccttctatgtcaagataacgaaagcccgtggtatcagctggcttcattctattccattctattttggctgttgcagaaaaacattcttctgttccactgccttctgttcacagtctgtcagctcgaaacgtctcttcaacagaggggtccagcaggcccatgctggagtcacttaacatgttgagtccgtccaggctcaggggttcaatctgcagctcctcttccagtggaaatggagtgtccacgttcaggctgacctcaggcaggcctgccagcgcactgttgaggtctttgaacaggctggtgctggagtcttctggcaggatggtgttcgggagactcccgcagttggaatacgggcttggtctcaaatgaaaagagtcctgcagttctcgggaaccttgttgcaccagaggcacctgttgaggaaaggcagggcctggcctcatggactgctggtcaaaacccacatctgggaagaagttggtcaaagatgagccctgggccgggagaagctgaaagtctgactgtggcagtgaggaggctgcctggggctgctgggcaggggcctcaggggcgcggggctgctgcaggaggggctgggtgagctcctggggtgcagggtaagggggtggcggcgacacctgggcttgagcttctgtgggcagaaaggaaagttggcttcggtctgaggacaccatctgggaggtaggatatggggccagtgggctggttgaagacagctgtctgctgaaaccttgatgtgcttcagggccaggagaaagcgtgagagggctgacgggaggctgccgacgccgagacgggccgctcaggtttgtggtggaaagagatgggttgctaagggaaaacagacggagcgaagggtgaagagcagatgcgttgggaacagatgtctgtgggtggttatttaaggaagaggaaagcacagtcttattgagcgtggcttggatggaggggttactccgagaactctggagaccagaggagcttcttatacccaggtgggtcatagcagctgggatgttgttcacactattccccacactcatactgccaaagtggtggtcggtggtgtccagggaggctggcaggggtgtcgagtagtggaggttggttagatctggcaatgaccctccagtgttcaaggtccccaagaagggtgagaggcctaggttttgaccattatgtggaaaagcattgccacctccaacatcacaggatcgagggcgtcctgacagggactgaatctccttggtctcccacagttgttttggcagtggcttcggaacatttaacagattctcttctttcaatgggccagggaaagatgctacttccccatgtccattattctcaccatcacagaaacccatgtatggggcaggccaggccgactggccccctcctccataggggtcctggggcttggtactcagagcactcgtgtgaagagcagaatcagaattggtcctgttaagtgcagatgtcagcctgaacccaggatgcttttcgtctttccaaggaggctgctgccttggccaactctcatccagaggctgtgaggaataattggctccaaaagcactaccatcaaattgtcgccctggcttgtccccagaccttcggtggagggggtggaagcggttcctggatggcctctccaccagcccgtgatggcgggttccccgaacattatcagcttggtgaaatgacggctgaaactctgacgcactgctccgcagctggctcacatttggtaaggatcctccatggtactgtgtaaggcgcagttgctgaagcttctgaaattgaacccgcgacagggtgaggtcggtcatgagctgctcgaaggcccgcgtctcctcggcctgtctctgcgtgtgcagcgcgatcttctcactgaacttccgcgggttggcgctgcccgagcccggcgaggcggccatggcgcggactctgcgcgggcagaagcgggagacggcggccgtggggcctgtacctcggcccacccgtccgtccacaggccgccggggccgccgcccgaagccagtcgtccggcgcgacccggcagaggagccgccgcggccccggagcc

SEQ ID NO: 18536 - RNA, 3920 nt, Homo sapiens
  source 1..3920: mol_type = other RNA
tgaggatatggcagggaaggggatagctacaggtgagcctgccttacggcatggcggacgcactcattcatcatgcgctgcacgcacggttctgcagcactcactccagcacacgactgtgctgccacgcacgtgttaggtgctacgggttcaacaatgataaggcactgtccctgccctcaaggagcttacggtctaggggggtgacattagactcccagcccacagagacacagctctggggagggatggggaagctcagttgctcggtgggtggggttagggcctcaccagctccctctggctgctcttagtggggaggtctgtgcttgtctggagtttgtctggaggccactgagtatgagacacctgcagtccctgtcttccttccccagcccccgaggaggagcacagttctcttcaggctcatcagtgccaggggactcttttcagtgactgataaaatggtcttcctcttcctctggtccataaggaaaaggtgtacttttctgaagcagcagaaaccagctgggagaaaatgaaaattagccttcagtctgcctaactcaagcctgccctcgggcttgtggtaaaaacttcatgtcgtaatccaggcgtgggagagagccgtggggtccactcagcctgggaatgtcccccgctggagggcctcgccctctgggtcaggtcagagcaggcatcgaggtgccctctccggtgccgccgccccaggccgagcctcccactccgggcccgccttcggtgcggacggagatcagtggttctgagcacactacacaatgctacggaggcctccagtgacacagtatttcctactcttacacatcggctgactggatggccagtaaaaagatgcagtggaggtgagctttccagttcatgggaagctccaagcagcctgcctgctgcaacacgactttggccacaggcgggagaggcagtacaaagctgtgtgatctggaggaagccacagtgtctgagatgggatctcatctgaaaccctggagccgtggcattgcttccttctatgtcaagataacgaaagcccgtggtatcagctggcttcattctattccattctattttggctgttgcagaaaaacattcttctgttccactgccttctgttcacagtctgtcagctcgaaacgtctcttcaacagaggggtccagcaggcccatgctggagtcacttaacatgttgagtccgtccaggctcaggggttcaatctgcagctcctcttccagtggaaatggagtgtccacgttcaggctgacctcaggcaggcctgccagcgcactgttgaggtctttgaacaggctggtgctggagtcttctggcaggatggtgttcgggagactcccgcagttggaatacgggcttggtctcaaatgaaaagagtcctgcagttctcgggaaccttgttgcaccagaggcacctgttgaggaaaggcagggcctggcctcatggactgctggtcaaaacccacatctgggaagaagttggtcaaagatgagccctgggccgggagaagctgaaagtctgactgtggcagtgaggaggctgcctggggctgctgggcaggggcctcaggggcgcggggctgctgcaggaggggctgggtgagctcctggggtgcagggtaagggggtggcggcgacacctgggcttgagcttctgtgggcagaaaggaaagttggcttcggtctgaggacaccatctgggaggtaggatatggggccagtgggctggttgaagacagctgtctgctgaaaccttgatgtgcttcagggccaggagaaagcgtgagagggctgacgggaggctgccgacgccgagacgggccgctcaggtttgtggtggaaagagatgggttgctaagggaaaacagacggagcgaagggtgaagagcagatgcgttgggaacagatgtctgtgggtggttatttaaggaagaggaaagcacagtcttattgagcgtggcttggatggaggggttactccgagaactctggagaccagaggagcttcttatacccaggtgggtcatagcagctgggatgttgttcacactattccccacactcatactgccaaagtggtggtcggtggtgtccagggaggctggcaggggtgtcgagtagtggaggttggttagatctggcaatgaccctccagtgttcaaggtccccaagaagggtgagaggcctaggttttgaccattatgtggaaaagcattgccacctccaacatcacaggatcgagggcgtcctgacagggactgaatctccttggtctcccacagttgttttggcagtggcttcggaacatttaacagattctcttctttcaatgggccagggaaagatgctacttccccatgtccattattctcaccatcacagaaacccatgtatggggcaggccaggccgactggccccctcctccataggggtcctggggcttggtactcagagcactcgtgtgaagagcagaatcagaattggtcctgttaagtgcagatgtcagcctgaacccaggatgcttttcgtctttccaaggaggctgctgccttggccaactctcatccagaggctgtgaggaataattggctccaaaagcactggagtgttctgggaaggatggaggctataagagaaggtaccatctgctcgggctcaggaggaaacaggagccttgatggagtggggccctatcctgcaggcctgggctgggcagctcaaataaatacagaatatggatcttttcttatccctctgtgcactcctttccgcccctttgccttccgtcctgatgttccctggggtcctgtggcctcgcagcctcaggccacacctgcctgcattgctctgagaggcaaaggatgctctcaggatccctgggcaccaggcagagtgtgagcaggtggagggggtggcgggagcctccgggcacaggagctttaggaggcgcttcctaagagcctcagggccagtgcccgtcttcctggtagagagcccctgtcctccatgctcgccttggccaatcgcatccttccctcggccccactgtcacccacagtccagtaactcataaatcgacacctccagctcccaacagttcttttgtgaactccaagtgcatacttccaactgcctactcaagttctctgccaaaagtacccaagacagctcaaattctaccaaaaatccaaccaatcactgtccccttaatctgttcctcttcttatagtccatctcatttagtgaggccaccgtccaccaagacactcatgttaggatctcagagtcatcccagtgtgttctctctctccccaagcctctgcagttctgtgcaggaaaatcttcctcctcgagttactgcctcaatccatcaacacagggactgctgttcctctcaacctgtggagtgttagagggaacagttcttactcttcaccaaaggaaggggagcagctcttcttcttctgataagagaggacatcagttggccagtttaccagtgggtggggttactgagccacagaagctgaaaacaagacccgccctggccctttctttgtgctgcttgacctgcggctgggtgagcaggcccagggttcccttctcttggcttcccgtccctgtgcggtcagtgtacctgggcagggctcaggaactgccttgtcggggcagcctggaagccagtcatttctctcctgctctggaactctgtgttctgccagggacacagtttgtggggcaggcctgagaccttccatgtagctggtggggtaagtgggctcggagtctggttaacagaacccacctaccaagacaagtttcagggtcagatttaatatataaaactggccacaatttggctccttcctgatt

SEQ ID NO: 18537 - RNA, 3119 nt, Homo sapiens
  source 1..3119: mol_type = other RNA
tgaggatatggcagggaaggggatagctacaggtgagcctgccttacggcatggcggacgcactcattcatcatgcgctgcacgcacggttctgcagcactcactccagcacacgactgtgctgccacgcacgtgttaggtgctacgggttcaacaatgataaggcactgtccctgccctcaaggagcttacggtctaggggggtgacattagactcccagcccacagagacacagctctggggagggatggggaagctcagttgctcggtgggtggggttagggcctcaccagctccctctggctgctcttagtggggaggtctgtgcttgtctggagtttgtctggaggccactgagtatgagacacctgcagtccctgtcttccttccccagcccccgaggaggagcacagttctcttcaggctcatcagtgccaggggactcttttcagtgactgataaaatggtcttcctcttcctctggtccataaggaaaaggtgtacttttctgaagcagcagaaaccagctgggagaaaatgaaaattagccttcagtctgcctaactcaagcctgccctcgggcttgtggtaaaaacttcatgtcgtaatccaggcgtgggagagagccgtggggtccactcagcctgggaatgtcccccgctggagggcctcgccctctgggtcaggtcagagcaggcatcgaggtgccctctccggtgccgccgccccaggccgagcctcccactccgggcccgccttcggtgcggacggagatcagtggttctgagcacactacacaatgctacggaggcctccagtgacacagtatttcctactcttacacatcggctgactggatggccagtaaaaagatgcagtggaggtgagctttccagttcatgggaagctccaagcagcctgcctgctgcaacacgactttggccacaggcgggagaggcagtacaaagctgtgtgatctggaggaagccacagtgtctgagatgggatctcatctgaaaccctggagccgtggcattgcttccttctatgtcaagataacgaaagcccgtggtatcagctggcttcattctattccattctattttggctgttgcagaaaaacattcttctgttccactgccttctgttcacagtctgtcagctcgaaacgtctcttcaacagaggggtccagcaggcccatgctggagtcacttaacatgttgagtccgtccaggctcaggggttcaatctgcagctcctcttccagtggaaatggagtgtccacgttcaggctgacctcaggcaggcctgccagcgcactgttgaggtctttgaacaggctggtgctggagtcttctggcaggatggtgttcgggagactcccgcagttggaatacgggcttggtctcaaatgaaaagagtcctgcagttctcgggaaccttgttgcaccagaggcacctgttgaggaaaggcagggcctggcctcatggactgctggtcaaaacccacatctgggaagaagttggtcaaagatgagccctgggccgggagaagctgaaagtctgactgtggcagtgaggaggctgcctggggctgctgggcaggggcctcaggggcgcggggctgctgcaggaggggctgggtgagctcctggggtgcagggtaagggggtggcggcgacacctgggcttgagcttctgtgggcagaaaggaaagttggcttcggtctgaggacaccatctgggaggtaggatatggggccagtgggctggttgaagacagctgtctgctgaaaccttgatgtgcttcagggccaggagaaagcgtgagagggctgacgggaggctgccgacgccgagacgggccgctcaggtttgtggtggaaagagatgggttgctaagggaaaacagacggagcgaagggtgaagagcagatgcgttgggaacagatgtctgtgggtggttatttaaggaagaggaaagcacagtcttattgagcgtggcttggatggaggggttactccgagaactctggagaccagaggagcttcttatacccaggtgggtcatagcagctgggatgttgttcacactattccccacactcatactgccaaagtggtggtcggtggtgtccagggaggctggcaggggtgtcgagtagtggaggttggttagatctggcaatgaccctccagtgttcaaggtccccaagaagggtgagaggcctaggttttgaccattatgtggaaaagcattgccacctccaacatcacaggatcgagggcgtcctgacagggactgaatctccttggtctcccacagttgttttggcagtggcttcggaacatttaacagattctcttctttcaatgggccagggaaagatgctacttccccatgtccattattctcaccatcacagaaacccatgtatggggcaggccaggccgactggccccctcctccataggggtcctggggcttggtactcagagcactcgtgtgaagagcagaatcagaattggtcctgttaagtgcagatgtcagcctgaacccaggatgcttttcgtctttccaaggaggctgctgccttggccaactctcatccagaggctgtgaggaataattggctccaaaagcactggagtgttctgggaaggatggaggctataagagaaggtaccatctgctcgggctcaggaggaaacaggagccttgatggagtggggccctatcctgcaggcctgggctgggcagctcaaataaatacagaatctgggcagggctcaggaactgccttgtcggggcagcctggaagccagtcatttctctcctgctctggaactctgtgttctgccagggacacagtttgtggggcaggcctgagaccttccatgtagctggtggggtaagtgggctcggagtctggttaacagaacccacctaccaagacaagtttcagggtcagatttaatatataaaactggccacaatttggctccttcctgattgctcagccatgtgtttattgtcattctacttctttttgtccctttacctctaactatgtcccactagaagacatcttaaagtgaaactgtaagggaggatat

SEQ ID NO: 18538 - RNA, 3163 nt, Homo sapiens
  source 1..3163: mol_type = other RNA
tgaggatatggcagggaaggggatagctacaggtgagcctgccttacggcatggcggacgcactcattcatcatgcgctgcacgcacggttctgcagcactcactccagcacacgactgtgctgccacgcacgtgttaggtgctacgggttcaacaatgataaggcactgtccctgccctcaaggagcttacggtctaggggggtgacattagactcccagcccacagagacacagctctggggagggatggggaagctcagttgctcggtgggtggggttagggcctcaccagctccctctggctgctcttagtggggaggtctgtgcttgtctggagtttgtctggaggccactgagtatgagacacctgcagtccctgtcttccttccccagcccccgaggaggagcacagttctcttcaggctcatcagtgccaggggactcttttcagtgactgataaaatggtcttcctcttcctctggtccataaggaaaaggtgtacttttctgaagcagcagaaaccagctgggagaaaatgaaaattagccttcagtctgcctaactcaagcctgccctcgggcttgtggtaaaaacttcatgtcgtaatccaggcgtgggagagagccgtggggtccactcagcctgggaatgtcccccgctggagggcctcgccctctgggtcaggtcagagcaggcatcgaggtgccctctccggtgccgccgccccaggccgagcctcccactccgggcccgccttcggtgcggacggagatcagtggttctgagcacactacacaatgctacggaggcctccagtgacacagtatttcctactcttacacatcggctgactggatggccagtaaaaagatgcagtggaggtgagctttccagttcatgggaagctccaagcagcctgcctgctgcaacacgactttggccacaggcgggagaggcagtacaaagctgtgtgatctggaggaagccacagtgtctgagatgggatctcatctgaaaccctggagccgtggcattgcttccttctatgtcaagataacgaaagcccgtggtatcagctggcttcattctattccattctattttggctgttgcagaaaaacattcttctgttccactgccttctgttcacagtctgtcagctcgaaacgtctcttcaacagaggggtccagcaggcccatgctggagtcacttaacatgttgagtccgtccaggctcaggggttcaatctgcagctcctcttccagtggaaatggagtgtccacgttcaggctgacctcaggcaggcctgccagcgcactgttgaggtctttgaacaggctggtgctggagtcttctggcaggatggtgttcgggagactcccgcagttggaatacgggcttggtctcaaatgaaaagagtcctgcagttctcgggaaccttgttgcaccagaggcacctgttgaggaaaggcagggcctggcctcatggactgctggtcaaaacccacatctgggaagaagttggtcaaagatgagccctgggccgggagaagctgaaagtctgactgtggcagtgaggaggctgcctggggctgctgggcaggggcctcaggggcgcggggctgctgcaggaggggctgggtgagctcctggggtgcagggtaagggggtggcggcgacacctgggcttgagcttctgtgggcagaaaggaaagttggcttcggtctgaggacaccatctgggaggtaggatatggggccagtgggctggttgaagacagctgtctgctgaaaccttgatgtgcttcagggccaggagaaagcgtgagagggctgacgggaggctgccgacgccgagacgggccgctcaggtttgtggtggaaagagatgggttgctaagggaaaacagacggagcgaagggtgaagagcagatgcgttgggaacagatgtctgtgggtggttatttaaggaagaggaaagcacagtcttattgagcgtggcttggatggaggggttactccgagaactctggagaccagaggagcttcttatacccaggtgggtcatagcagctgggatgttgttcacactattccccacactcatactgccaaagtggtggtcggtggtgtccagggaggctggcaggggtgtcgagtagtggaggttggttagatctggcaatgaccctccagtgttcaaggtccccaagaagggtgagaggcctaggttttgaccattatgtggaaaagcattgccacctccaacatcacaggatcgagggcgtcctgacagggactgaatctccttggtctcccacagttgttttggcagtggcttcggaacatttaacagattctcttctttcaatgggccagggaaagatgcttccccatgtccattattctcaccatcacagaaacccatgtatggggcaggccaggccgactggccccctcctccataggggtcctggggcttggtactcagagcactcgtgtgaagagcagaatcagaattggtcctgttaagtgcagatgtcagcctgaacccaggatgcttttcgtctttccaaggaggctgctgccttggccaactctcatccagaggctgtgaggaataattggctccaaaagcactaccatcaaattgtcgccctggcttgtccccagaccttcggtggagggggtggaagcggttcctggatggcctctccaccagcccgtgatggcgggttccccgaacattatcagcttggtgaaatgacggctgaaactctgacgcactgctccgcagctggctcacatttggtaaggatcctccatggtactgtgtaaggcgcagttgctgaagcttctgaaattgaacccgcgacagggtgaggtcggtcatgagctgctcgaaggcccgcgtctcctcggcctgtctctgcgtgtgcagcgcgatcttctcactgaacttccgcgggttggcgctgcccgagcccggcgaggcggccatggcgcggactctgcgcgggcagaagcgggagacggcggccgtggggcctgtacctcggcccacccgtccgtccacaggccgccggggccgccgcccgaagccagtcgtccggcgcgacccggcagaggagccgccgcggccccggagccagcgagcg

SEQ ID NO: 18539 - RNA, 203 nt, Homo sapiens
  source 1..203: mol_type = other RNA
tgaggcccttggggcacagtggtgaaacctgcaaggaacatacccagagagctggcggctgcaggtggccagggcgggcaatgctctgcatcttgtcagcagcccttccatgacaccctggcaccgggaagcacaggcaccgcaatcccagcccacgcctcccgcaagaccaccgccgtgccgggccagcgcgcttgcgcctc

SEQ ID NO: 18540 - RNA, 1015 nt, Homo sapiens
  source 1..1015: mol_type = other RNA
tgagggacccaggacaggagatgagctcatctgcaacagtctcatgagccttggcaatctgccctagctcctgtatcaagccctggaagcagtccttacggagcaaatgctggcaggataggagatgagagcccatacctggcaggtcctgatggcacaatgagcaggtcattaccatggcctccatctgtccactcttagggcagtgtttctggccagctagtggcagccccataaagctcatgcccatgtccacagccatgcctgtgcccaggactggggcttttccactgatatcctcaggtgagaagcagcgtgtagagcgagccagctccactccctgggaccaaaaagagagtctagccatctctgccgtggaaaacaaagcgtggaggtgtctgctgtttgtctgaaggcgaacaaacccttcaaaagtgtcccgtacctgtgcctctccttattggtagacaagcttgacctgtttctgcagtcaatctgttatatgttgttttgttcacagtatatgaggaaaatccagtctcacacagacatacagcatataatccagcagtctcacttctgggaatttatcctccattgacagatcatcttcccaaggttaggttccaggtaacccagctcatttcttgtgcacttactggccagttttgatgtcaaatagacgacgatgtcttctttgatctcccctcctattctcaagacccctcttcctgctggtcacatgcagtatgtgattaaggttgatggagggatgaagaccataatgctgaccacctatgcagcgtctgacaagtcacccaattcttctgtgcttcagttttcacacacgtaaaatgaggctggtagtgctgtaccttcaggcagatgtattttgtaaattgccaagtgctctgaaaatgttggttgttatccttgtggactgaagtgttcgaaaccgtacaccgccaccaggacactccgtgatgggggatcaccaccctcagaaagaggaagc

SEQ ID NO: 18541 - RNA, 1415 nt, Homo sapiens
  source 1..1415: mol_type = other RNA
tgagggacccaggacaggagatgagctcatctgcaacagtctcatgagccttggcaatctgccctagctcctgtatcaagccctggaagcagtccttacggagcaaatgctggcaggataggagatgagagcccatacctggcaggtcctgatggcacaatgagcaggtcattaccatggcctccatctgtccactcttagggcagtgtttctggccagctagtggcagccccataaagctcatgcccatgtccacagccatgcctgtgcccaggactggggcttttccactgatatcctcaggtgagaagcagcgtgtagagcgagccagctccactccctgggaccaaaaagagagtctagccatctctgccgtggaaaacaaagcgtggaggtgtctgctgtttgtctgaaggcgaacaaacccttcaaaagtgtcccgtacctgtgcctctccttattggtagacaagcttgacctgtttctgcagtcaatctgttatatgttgttttgttcacagtatatgaggaaaatccagtctcacacagacatacagcatataatccagcagtctcacttctgggaatttatcctccattgacagatcatcttcccaaggttaggttccaggtaacccagctcatttcttgtgcacttactggccagttttgatgtcaaatagacgacgatgtcttctttgatctcccctcctattctcaagacccctcttcctgctggtcacatgcagtatgtgattaaggttgatggagggatgaagaccataatgctgaccacctatgcagcgtctgacaagtcacccaattcttctgtgcttcagttttcacacacgtaaaatgaggctggtagtgctgtaccttcaggcagatgtattttgtaaattgccaagtgctctgaaaatgttggttgttatccttgtggactgaagtgttctcgcgagacttggcgaaggccttcctttttcgtctgggctgccaacatggtaggtgtttcgtttcttgcctcctcttccttgccggcggagacccctaagctgtattcccattgcccctagtcatccactccctaccatggtcggggcttccaggctgcgcatggccgcctgcggggcagggtggccggcgcgggcccggggcggggctcccggagccgtgtgttaggcccgcggttcggatctctaggacacgcgggcccctgcgctaccgtggtgagacctcacggccctgagcggatcggtaccctcagctttcccaaacgctccagaagttaggtctttgacccacaggcttacaggaccatctcggctggcgggcatcgccccctgcccctaattccttaggccttaccaccaagctttttccacacagccatccagactgaggaagacccggaaactt

SEQ ID NO: 18542 - RNA, 972 nt, Homo sapiens
  source 1..972: mol_type = other RNA
tgagggacccaggacaggagatgagctcatctgcaacagtctcatgagccttggcaatctgccctagctcctgtatcaagccctggaagcagtccttacggagcaaatgctggcaggataggagatgagagcccatacctggcaggtcctgatggcacaatgagcaggtcattaccatggcctccatctgtccactcttagggcagtgtttctggccagctagtggcagccccataaagctcatgcccatgtccacagccatgcctgtgcccaggactggggcttttccactgatatcctcaggtgagaagcagcgtgtagagcgagccagctccactccctgggaccaaaaagagagtctagccatctctgccgtggaaaacaaagcgtggaggtgtctgctgtttgtctgaaggcgaacaaacccttcaaaagtgtcccgtacctgtgcctctccttattggtagacaagcttgacctgtttctgcagtcaatctgttatatgttgttttgttcacagtatatgaggaaaatccagtctcacacagacatacagctccattgacagatcatcttcccaaggttaggttccaggtaacccagctcatttcttgtgcacttactggccagttttgatgtcaaatagacgacgatgtcttctttgatctcccctcctattctcaagacccctcttcctgctggtcacatgcagtatgtgattaaggttgatggagggatgaagaccataatgctgaccacctatgcagcgtctgacaagtcacccaattcttctgtgcttcagttttcacacacgtaaaatgaggctggtagtgctgtaccttcaggcagatgtattttgtaaattgccaagtgctctgaaaatgttggttgttatccttgtggactgaagtgttcgaaaccgtacaccgccaccaggacactccgtgatgggggatcaccaccctcagaaag

SEQ ID NO: 18543 - RNA, 979 nt, Homo sapiens
  source 1..979: mol_type = other RNA
tgagggacccaggacaggagatgagctcatctgcaacagtctcatgagccttggcaatctgccctagctcctgtatcaagccctggaagcagtccttacggagcaaatgctggcaggataggagatgagagcccatacctggcaggtcctgatggcacaatgagcaggtcattaccatggcctccatctgtccactcttagggcagtgtttctggccagctagtggcagccccataaagctcatgcccatgtccacagccatgcctgtgcccaggactggggcttttccactgatatcctcaggtgagaagcagcgtgtagagcgagccagctccactccctgggaccaaaaagagagtctagccatctctgccgtggaaaacaaagcgtggaggtgtctgctgtttgtctgaaggcgaacaaacccttcaaaagtgtcccgtacctgtgcctctccttattggtagacaagcttgacctgtttctgcagtcaatctgttatatgttgttttgttcacagtatatgaggaaaatccagtctcacacagacatacagctccattgacagatcatcttcccaaggttaggttccaggtaacccagctcatttcttgtgcacttactggccagttttgatgtcaaatagacgacgatgtcttctttgatctcccctcctattctcaagacccctcttcctgctggtcacatgcagtatgtgattaaggttgatggagggatgaagaccataatgctgaccacctatgcagcgtctgacaagtcacccaattcttctgtgcttcagttttcacacacgtaaaatgaggctggtagtgctgtaccttcaggcagatgtattttgtaaattgccaagtgctctgaaaatgttggttgttatccttgtggactgaagtgttcgaaaccgtacaccgccaccaggacactccgtgatgggggatcaccaccctcagaaagaggaagc

SEQ ID NO: 18544 - RNA, 1365 nt, Homo sapiens
  source 1..1365: mol_type = other RNA
tgagggacccaggacaggagatgagctcatctgcaacagtctcatgagccttggcaatctgccctagctcctgtatcaagccctggaagcagtccttacggagcaaatgctggcaggataggagatgagagcccatacctggcaggtcctgatggcacaatgagcaggtcattaccatggcctccatctgtccactcttagggcagtgtttctggccagctagtggcagccccataaagctcatgcccatgtccacagccatgcctgtgcccaggactggggcttttccactgatatcctcaggtgagaagcagcgtgtagagcgagccagctccactccctgggaccaaaaagagagtctagccatctctgccgtggaaaacaaagcgtggaggtgtctgctgtttgtctgaaggcgaacaaacccttcaaaagtgtcccgtacctgtgcctctccttattggtagacaagcttgacctgtttctgcagtcaatctgttatatgttgttttgttcacagtatatgaggaaaatccagtctcacacagacatacagctccattgacagatcatcttcccaaggttaggttccaggtaacccagctcatttcttgtgcacttactggccagttttgatgtcaaatagacgacgatgtcttctttgatctcccctcctattctcaagacccctcttcctgctggtcacatgcagtatgtgattaaggttgatggagggatgaagaccataatgctgaccacctatgcagcgtctgacaagtcacccaattcttctgtgcttcagttttcacacacgtaaaatgaggctggtagtgctgtaccttcaggcagatgtattttgtaaattgccaagtgctctgaaaatgttggttgttatccttgtggactgaagtgttctcgcgagacttggcgaaggccttcctttttcgtctgggctgccaacatggtaggtgtttcgtttcttgcctcctcttccttgccggcggagacccctaagctgtattcccattgcccctagtcatccactccctaccatggtcggggcttccaggctgcgcatggccgcctgcggggcagggtggccggcgcgggcccggggcggggctcccggagccgtgtgttaggcccgcggttcggatctctaggacacgcgggcccctgcgctaccgtggtgagacctcacggccctgagcggatcggtaccctcagctttcccaaacgctccagaagttaggtctttgacccacaggcttacaggaccatctcggctggcgggcatcgccccctgcccctaattccttaggccttaccaccaagctttttccacacagccatccagactgagga

SEQ ID NO: 18545 - RNA, 993 nt, Homo sapiens
  source 1..993: mol_type = other RNA
tgagggacccaggacaggagatgagctcatctgcaacagtctcatgagccttggcaatctgccctagctcctgtatcaagccctggaagcagtccttacggagcaaatgctggcaggataggagatgagagcccatacctggcaggtcctgatggcacaatgagcaggtcattaccatggcctccatctgtccactcttagggcagtgtttctggccagctagtggcagccccataaagctcatgcccatgtccacagccatgcctgtgcccaggactggggcttttccactgatatcctcaggtgagaagcagcgtgtagagcgagccagctccactccctgggaccaaaaagagagtctagccatctctgccgtggaaaacaaagcgtggaggtgtctgctgtttgtctgaaggcgaacaaacccttcaaaagtgtcccgtacctgtgcctctccttattggtagacaagcttgacctgtttctgcagtcaatctgttatatgttgttttgttcacagtatatgaggaaaatccagtctcacacagacatacagtggccagttttgatgtcaaatagacgacgatgtcttctttgatctcccctcctattctcaagacccctcttcctgctggtcacatgcagtatgtgattaaggttgatggagggatgaagaccataatgctgaccacctatgcagcgtctgacaagtcacccaattcttctgtgcttcagttttcacacacgtaaaatgaggctggtagtgctgtaccttcaggcagatgtattttgtaaattgccaagtgctctgaaaatgttggttgttatccttgtggactgaagtgttcgaaaccgtacaccgccaccaggacactccgtgatgggggatcaccaccctcagaaagaggaagcgactagcaggcgcgcaatcccgcgagaccaggaggccccgcccgaagcccggcctctgtgaccggaagtgaggcgttttgc

SEQ ID NO: 18546 - RNA, 177 nt, Homo sapiens
  source 1..177: mol_type = other RNA
tgagggacccaggacaggagatgagctcgcatcattttaaaaaacagcaggagcccaagatatccctccatgcccccggcactgaaggagggtgtgggggggccttcaacagacattgaaatctgtctcctacatactcacctgctcctgccacttcacctgaagtccttatcctgt

SEQ ID NO: 18547 - RNA, 479 nt, Homo sapiens
  source 1..479: mol_type = other RNA
tgagggacccaggacaggagatgagctctcagcctcctaaagtgctgggattacaggcatgagccactgtgcctggcagaggactgcatttttcgggagtttgtgtgttccatgtgtactccttgcactcacagcactgaaagtagtaagaagccacctggaagttttctggaaaaaaagccagtgcaggtttataaggaaagcagaggtgtggggcttgggaaaagcttttaattaaaaaatatgagttctaggcccagggctggcagtatctaactatgtaaccttgggtaagtcaccccctttcactcaaccttactttctacaccattaaaatgagggaataggaatgcaggggagtacaaattatccaacccatttactctgcctacagcagccagacgtttttttttcctggaggccaggcacggtggctcatgcctgtaatcccaacattttggaatgccaaggcaggagga

SEQ ID NO: 18548 - RNA, 1439 nt, Homo sapiens
  source 1..1439: mol_type = other RNA
tgagggacccaggacaggagatgagctctgagatactcctgcaagaaagagcttggttgactcctcctgtttctgtttatctcgaaggctctgcagcaattttcccaaactgaacagcaagagggagacctcaaagaggcgactctcttcctagctgcatctccttcctaatcctctgggtgccttggaatagaagctcagaaggaagaaaacgacattttcaactttcaggaactagctctgtcgccctctgcacagctcgggagacagcactctcagccttttaggactccatccaaaaatccttcagccctccatgttccccaaaatgacagtgctcatgtgtggctggaacctgccccgatccggcagctcatttaaatagagctcatcacaacaacagtgttggtggtgaagtgagtagctgcaggaccctggggaccccctgtttatacgtaggaagaatgatgcaatctgggtatcaaaatagcaatccagaatggaataacaggctcacgcagcagcggtgcctgcacagccagagctcaagttgacacactctgtcagccccacactgctgcagcacgcagatgccaggcacacactctcaccgcatcattttaaaaaacagcaggagcccaagatatccctccatgcccccggcactgaaggagggtgtgggggggccttcaacagacattgaaatctgtctcctacatactcacctgctcctgccacttcacctgaagtccttatcctgtgacgtcacagtcagttgccatagtgaccaattgtccgtcacaagcagaggattaggacttcggatggagaagacacacatttacgatgcacaaaggtcctgggaggtctcccttggcagttaactctacccaccaggaagatccagtcacacacaagcagggagggaaaaagggaagaatgaacagggttgactggaggagacattaggatggggcaagactacaagtacagcataatttcaaaagcacagagcaaccagatgagggggagtggcagggatgtgcttggaaagaccggaaggagagtaagctcctgaagggacctgaatgctaagctcaggagcttgaccttcatcctaaaataaaaggcagcccaaaaagtttctggagagtgactgagctgggctttatgattatcttgatggactgaacacagggaggtcagggtagttgagcattaatgggaccctaaataagggtaaaaatggaaaaaagcaaaagaagactcatttcaaagagaactgacaggacacaagcaaattaggatgttggggctagtggtggtgtgtgaagaacaaggaatcaagtggaggggctgtcatgaacagaggtaggtaacaggaggaagagagcagtggccaaatctcatgttatctataccttcctttctctggcatc

SEQ ID NO: 18549 - RNA, 868 nt, Homo sapiens
  source 1..868: mol_type = other RNA
tgagggacccaggacaggagatgagctctggcaggtcctgatggcacaatgagcaggtcattaccatggcctccatctgtccactcttagggcagtgtttctggccagctagtggcagccccataaagctcatgcccatgtccacagccatgcctgtgcccaggactggggcttttccactgatatcctcaggtgagaagcagcgtgtagagcgagccagctccactccctgggaccaaaaagagagtctagccatctctgccgtggaaaacaaagcgtggaggtgtctgctgtttgtctgaaggcgaacaaacccttcaaaagtgtcccgtacctgtgcctctccttattggtagacaagcttgacctgtttctgcagtcaatctgttatatgttgttttgttcacagtatatgaggaaaatccagtctcacacagacatacagctccattgacagatcatcttcccaaggttaggttccaggtaacccagctcatttcttgtgcacttactggccagttttgatgtcaaatagacgacgatgtcttctttgatctcccctcctattctcaagacccctcttcctgctggtcacatgcagtatgtgattaaggttgatggagggatgaagaccataatgctgaccacctatgcagcgtctgacaagtcacccaattcttctgtgcttcagttttcacacacgtaaaatgaggctggtagtgctgtaccttcaggcagatgtattttgtaaattgccaagtgctctgaaaatgttggttgttatccttgtggactgaagtgttcgaaaccgtacaccgccaccaggacactccgtgatgggggatcaccaccctcagaaagaggaagc

SEQ ID NO: 18550 - RNA, 2321 nt, Homo sapiens
  source 1..2321: mol_type = other RNA
tgagggacccaggacaggagatgagctctgtgtccagggatgagggtgatctggaaaggggttggctatggcagtgaatgcagcagtaccgctacaatctcctctgtctcatctcttcaaaatacgaaagaatgatatgatggcagttgctccagacttatagtcagacaaatgtaagtccaaaataccaggcctaccagccaatgaccttgggcaaaacacttaatctcacttaattgccctgtaccccagtttcttcatatgtaaaatagggaaaataagagttgctgtgcacattaaattagataagacttcagaaatcacatggtcctccatgaatgtcaactttggagttcaaaagattcctcatatcctattcacagtaatgcaataaactcaattaccaactctctggtgacgaaagttagtttgagtggtagattcaaaaaatggccacaaattcttcccctccctgcatccatacccttgcaatcctaccatcaaaaggtaagactctccacgagcttcaggtcagtgatgagtttttaatttttaaaagaggtaggaccctttgccctttgaatctaagctcaccttgtgactttctttggccaacagaatgcagcaaaagtgacaagttttccaagcctagacctcagtggccttatataattctgctcttgttcttagaactttaagagtgccatgtgaaaaatctaacctggcattgagactgctggaagatgagagatcatgcagagaaagttctcagttgtctcaggcatcccacctgaggccatcatagaccagccagccccaactaacccactagctgaatacagtgcaagagtgaacacagttataattagctaagcccaggccaaaccagaagaattacccagagaatcccagcccaaacagccaaactgtagaatcataaaataaataaagtttagttgttttaagcacaaagtttagaggtggcttgttatgcagtaaaagctaactgatacatcccaggaaaatagaaatccacaaaatcatgaaaaataatagtttaatactccctcaccccaccaaaaaaaaaaagaaaagaaaagaaaagaaaaactttctgagtttttgcagagccatgggtgttaatgacaggactgtatctggaatgtcctgcatattctcctgcctgtcaagaacaatggccagaggtggagaaggatgctctccacaggtgacatcatccaggggaataaggctactgtccctctcttccacttggctcaccctgaggtgacctcctcatctacagcaggacagaaatgctgctctaattgttgaaaacgacttccacaagacatcccgggtaccagatgcccaaacatcagtcattgtaacatggcctcacgagcagaatgaaaaaagagaaagaactgaataggtcaaacaaggcctcatcacacatcctctgctcccttggccttaaagccaaagtcctcagcttggcattcaatgccccttgtaaattgaccttatctctctctaatctcatctttagctttgcctaacatacaacctgtgtttttgccatgcccaacatctctgctatctcttgaatacaccagacttttgcatgactctgtgtctgtgaaaaatgctgtttcctcttcctgaaatactctttcttgcccctctccttttcagataaactcctattcatcctttcatacctgttcaaatgttccacctttgagcagcaagatcaatttcccccgggatgagttaattagtccctcttctgggttcccgcagcaccctgaacatccttccagtacaacgaatatcacattgcattttaaatacctgttcatatgtctcagcctcctaaagtgctgggattacaggcatgagccactgtgcctggcagaggactgcatttttcgggagtttgtgtgttccatgtgtactccttgcactcacagcactgaaagtagtaagaagccacctggaagttttctggaaaaaaagccagtgcaggtttataaggaaagcagaggtgtggggcttgggaaaagcttttaattaaaaaatatgagttctaggcccagggctggcagtatctaactatgtaaccttgggtaagtcaccccctttcactcaaccttactttctacaccattaaaatgagggaataggaatgcaggggagtacaaattatccaacccatttactctgcctacagcagccagacgtttttttttcctggaggccaggcacggtggctcatgcctgtaatcccaacattttggaatgccaaggcaggagga

SEQ ID NO: 18551 - RNA, 1725 nt, Homo sapiens
  source 1..1725: mol_type = other RNA
tgagggacccaggacaggagatgagctctgttcaaatgttccacctttgagcagcaagatcaatttcccccgggatgagttaattagtccctcttctgggttcccgcagcaccctgaacatccttccagtacaacgaatatcacattgcattttaaatacctgttcatatgtctcagcctcctaaagtgctgggattacaggcatgagccactgtgcctggcagaggactgcatttttcgggagtttgtgtgttccatgtgtactccttgcactcacagcactgaaagtagtaagaagccacctggaagttttctgagatactcctgcaagaaagagcttggttgactcctcctgtttctgtttatctcgaaggctctgcagcaattttcccaaactgaacagcaagagggagacctcaaagaggcgactctcttcctagctgcatctccttcctaatcctctgggtgccttggaatagaagctcagaaggaagaaaacgacattttcaactttcaggaactagctctgtcgccctctgcacagctcgggagacagcactctcagccttttaggactccatccaaaaatccttcagccctccatgttccccaaaatgacagtgctcatgtgtggctggaacctgccccgatccggcagctcatttaaatagagctcatcacaacaacagtgttggtggtgaagtgagtagctgcaggaccctggggaccccctgtttatacgtaggaagaatgatgcaatctgggtatcaaaatagcaatccagaatggaataacaggctcacgcagcagcggtgcctgcacagccagagctcaagttgacacactctgtcagccccacactgctgcagcacgcagatgccaggcacacactctcaccgcatcattttaaaaaacagcaggagcccaagatatccctccatgcccccggcactgaaggagggtgtgggggggccttcaacagacattgaaatctgtctcctacatactcacctgctcctgccacttcacctgaagtccttatcctgtgacgtcacagtcagttgccatagtgaccaattgtccgtcacaagcagaggattaggacttcggatggagaagacacacatttacgatgcacaaaggtcctgggaggtctcccttggcagttaactctacccaccaggaagatccagtcacacacaagcagggagggaaaaagggaagaatgaacagggttgactggaggagacattaggatggggcaagactacaagtacagcataatttcaaaagcacagagcaaccagatgagggggagtggcagggatgtgcttggaaagaccggaaggagagtaagctcctgaagggacctgaatgctaagctcaggagcttgaccttcatcctaaaataaaaggcagcccaaaaagtttctggagagtgactgagctgggctttatgattatcttgatggactgaacacagggaggtcagggtagttgagcattaatgggaccctaaataagggtaaaaatggaaaaaagcaaaagaagactcatttcaaagagaactgacaggacacaagcaaattaggatgttggggctagtggtggtgtgtgaagaacaaggaatcaagtggaggggctgtcatgaacagaggtaggtaacaggaggaagagagcagtggccaaatctcatgttatctataccttcctttctctggcatc

SEQ ID NO: 18552 - RNA, 403 nt, Homo sapiens
  source 1..403: mol_type = other RNA
tgagggacccaggacaggagatgagctctgttcaaatgttccacctttgagcagcaagatcaatttcccccgggatgagttaattagtccctcttctgggttcccgcagcaccctgaacatccttccagtacaacgaatatcacattgcattttaaatacctgttcatatgtctcagcctcctaaagtgctgggattacaggcatgagccactgtgcctggcagaggactgcatttttcgggagtttgtgtgttccatgtgtactccttgcactcacagcactgaaagtagtaagaagccacctggaagttttctggcaggtcctgatggcacaatgagcaggtcattaccatggcctccatctgtccactcttagggcagtgtttctggccagctagtggca

SEQ ID NO: 18553 - RNA, 403 nt, Homo sapiens
  source 1..403: mol_type = other RNA
tgagggacccaggacaggagatgagctctgttcaaatgttccacctttgagcagcaagatcaatttcccccgggatgagttaattagtccctcttctgggttcccgcagcaccctgaacatccttccagtacaacgaatatcacattgcattttaaatacctgttcatatgtctcagcctcctaaagtgctgggattacaggcatgagccactgtgcctggcagaggactgcatttttcgggagtttgtgtgttccatgtgtactccttgcactcacagcactgaaagtagtaagaagccacctggaagttttctttgctctggtccccatcattagcttttgaagatcttgcccagctggtctcctcagtacctgagaggtgacgcagacccatcttcctag

SEQ ID NO: 18554 - RNA, 1584 nt, Homo sapiens
  source 1..1584: mol_type = other RNA
tgagggacccaggacaggagatgagctctgttcaaatgttccacctttgagcagcaagatcaatttcccccgggatgagttaattagtccctcttctgggttcccgcagcaccctgaacatccttccagtacaacgaatatcacattgcattttaaatacctgttcatatgtctgagatactcctgcaagaaagagcttggttgactcctcctgtttctgtttatctcgaaggctctgcagcaattttcccaaactgaacagcaagagggagacctcaaagaggcgactctcttcctagctgcatctccttcctaatcctctgggtgccttggaatagaagctcagaaggaagaaaacgacattttcaactttcaggaactagctctgtcgccctctgcacagctcgggagacagcactctcagccttttaggactccatccaaaaatccttcagccctccatgttccccaaaatgacagtgctcatgtgtggctggaacctgccccgatccggcagctcatttaaatagagctcatcacaacaacagtgttggtggtgaagtgagtagctgcaggaccctggggaccccctgtttatacgtaggaagaatgatgcaatctgggtatcaaaatagcaatccagaatggaataacaggctcacgcagcagcggtgcctgcacagccagagctcaagttgacacactctgtcagccccacactgctgcagcacgcagatgccaggcacacactctcaccgcatcattttaaaaaacagcaggagcccaagatatccctccatgcccccggcactgaaggagggtgtgggggggccttcaacagacattgaaatctgtctcctacatactcacctgctcctgccacttcacctgaagtccttatcctgtgacgtcacagtcagttgccatagtgaccaattgtccgtcacaagcagaggattaggacttcggatggagaagacacacatttacgatgcacaaaggtcctgggaggtctcccttggcagttaactctacccaccaggaagatccagtcacacacaagcagggagggaaaaagggaagaatgaacagggttgactggaggagacattaggatggggcaagactacaagtacagcataatttcaaaagcacagagcaaccagatgagggggagtggcagggatgtgcttggaaagaccggaaggagagtaagctcctgaagggacctgaatgctaagctcaggagcttgaccttcatcctaaaataaaaggcagcccaaaaagtttctggagagtgactgagctgggctttatgattatcttgatggactgaacacagggaggtcagggtagttgagcattaatgggaccctaaataagggtaaaaatggaaaaaagcaaaagaagactcatttcaaagagaactgacaggacacaagcaaattaggatgttggggctagtggtggtgtgtgaagaacaaggaatcaagtggaggggctgtcatgaacagaggtaggtaacaggaggaagagagcagtggccaaatctcatgttatctataccttcctttctctggcatc

SEQ ID NO: 18555 - RNA, 261 nt, Homo sapiens
  source 1..261: mol_type = other RNA
tgagggacccaggacaggagatgagctctgttcaaatgttccacctttgagcagcaagatcaatttcccccgggatgagttaattagtccctcttctgggttcccgcagcaccctgaacatccttccagtacaacgaatatcacattgcattttaaatacctgttcatatgtctggcaggtcctgatggcacaatgagcaggtcattaccatggcctccatctgtccactcttagggcagtgtttctggccagctagtggc

SEQ ID NO: 18556 - RNA, 373 nt, Homo sapiens
  source 1..373: mol_type = other RNA
tgagggacccaggacaggagatgagctctgttcaaatgttccacctttgagcagcaagatcaatttcccccgggatgagttaattagtccctcttctgggttcccgcagcaccctgaacatccttccagtacaacgaatatcacattgcattttaaatacctgttcatatgtctttgctctggtccccatcattagcttttgaagatcttgcccagctggtctcctcagtacctgagaggtgacgcagacccatcttcctagttgctggggagaatctcagctaggctgtggcatctgcaacagtctcatgagccttggcaatctgccctagctcctgtatcaagccctggaagcagtccttacggagcaaat

SEQ ID NO: 18557 - RNA, 236 nt, Homo sapiens
  source 1..236: mol_type = other RNA
tgagggacccaggacaggagatgagctctttgctctggtccccatcattagcttttgaagatcttgcccagctggtctcctcagtacctgagaggtgacgcagacccatcttcctagttgctggggagaatctcagctaggctgtggcatctgcaacagtctcatgagccttggcaatctgccctagctcctgtatcaagccctggaagcagtccttacggagcaaatgctggcag

SEQ ID NO: 18558 - RNA, 190 nt, Homo sapiens
  source 1..190: mol_type = other RNA
tgagggacccaggacaggagatgagctctttgctctggtccccatcattagcttttgaagatcttgcccagctggtctcctcagtacctgagaggtgacgcagacccatcttcctagttgctggggagaatctcagctaggctgtggctgcactcccatgttcattgctgtattattcacaatagccagg

SEQ ID NO: 18559 - RNA, 234 nt, Homo sapiens
  source 1..234: mol_type = other RNA
tgagggacccaggacaggagatgagctctttgctctggtccccatcattagcttttgaagatcttgcccagctggtctcctcagtacctgagaggtgacgcagacccatcttcctagttgctggggagaatctcagctaggctgtggctggcaggtcctgatggcacaatgagcaggtcattaccatggcctccatctgtccactcttagggcagtgtttctggccagctagtg

SEQ ID NO: 18560 - RNA, 327 nt, Homo sapiens
  source 1..327: mol_type = other RNA
tgagggacccaggacaggagatgagctctttgctctggtccccatcattagcttttgaagatcttgcccagctggtctcctcagtacctgagaggtgacgcagacccatcttcctagttgctggggagaatctcagctaggctgtggctgtattaattaaagatttgcacttgatccagcaattcaaatactgagtatacaatagtcccccccttattcatgggggctactttccaagatgcctgaaacagtggatagtaccaaaccctatatatactatatttttcctatgcatacatacctatgataaagtttaatttgtaaatt

SEQ ID NO: 18561 - RNA, 75 nt, Homo sapiens
  source 1..75: mol_type = other RNA
tgagggacccaggacaggagatggtgtggtggaagccactcccgtggcagccccgtgatccggaaggatttatct

SEQ ID NO: 18562 - RNA, 2352 nt, Homo sapiens
  source 1..2352: mol_type = other RNA
tgagggaggaggttgggtaagaaagggggaaagtgggacatggaggtggggtgagccaccttccctggcggcgaccagcattccttggtggcaggacaccttggccctggagtctcgaagaggcctcccttggactctgtagcgaccacgggtcccacctcaagcctccttggctttaccttccccatcaaatagtcatgtgccctcctgccctgcccaaccccagagttcaagagagaaaaacattcattacgaacgccttttatccctggccaaatccaagcctctttacctcgctatatatatatagatatacatatttgtctcatcccacttccctctccaggtctagtgaaccatcaactccaaggctagagctgagcagacccctccagaaaggctcatctcccaaaaagcagccattccccacctggctcccgaggcgcatacttaataaagtcagtctaatctccgaacgcgatccttccccaaatacaaaaataacagagctgtggctggggctgtcatgttgcccgccccattgtgaatggcttcaaaactccctgaataaagataagagaggattgtgtacgttttcaacacaaatggtggaaagtaataaaataaacatcaaaggtgagctcccacctactagcggctccgtcgctttttgtgcaacaaaggcaggaaaaaggaggaaactcggcgtggcagggcagcgggctggaagtgcaccttcccggggccgaggcgcccgctccctggactaatgacgccgcgtggggatcacgccccgggcgccctggggtgaggaacggtcccccctttcgagattgtccgacactggtgccagtgaggtcacagcaaaagtcccaaaggaatattggaaagaaatggccgtgaaccggtttgttcttgcccccgcccccgggaacacgccctctccgtcgttcctgttgactgtcagatcccgggaaccaagcggcggagctcggcggcatctgaggcttccgcagggacacaagtgcaggcacagcccagcaccctgcgccagacacagccgccccaggggaagaggaggacgctgctgtcctcccgcaggagtcaccagccaggtaaagaaaaaggtaaagtaagacaaagaaaagtgaaagtcggagcccatttagtgagcaagagtaaaggtcatccaaaaaggcgcatacaatttcaagcccaggagtgcattcattaaaacaagaggaaaagacaagatggtccttgaaaggagctcataggaaggggcacagcacaaggctcccgaaagaggtcactgcaagtgtcctgcgcaatttctgttcagcacctctgcagtgacgacaggggtttgctttcgtaagcagcatcgttttcactactacagaagcacatacgccgcgtgcagcttaggcccgagcaaagtccctgctcccctagacccagtcccttcaggtgtccccctaggggaactgtggcgtgtccccccaaccaggcgcactcgcctaaactgcgtccccgaactccagggcgcagggagccctcgcgggctgcccggggctggggcccacacctgaacggaggagccggctggcggagcggccccgcgcgcgcacacacgcacactcacagacacgcgcaaacccacagcggcgcgcgcgctccccattggcgggaggaggaaggcggggccggccgacccaaaacaaacaacctgcgccagcgactttgccgccgcgctgcagtgtggcctccgcctggtgcgcgcccgttggggagctggggaactggggagccgccaccacctcggccacctcgttcccccaccccttgccgtccgcgctcaggccccgcccccgcggagccgccgcagggttatattgggccggcccgaaggtggaggcgagacgcagccgcggcaggccagcggggagatgctgccccggaggctgggagcgggaaggcggctgcgggcgcagcggcctcggggactcgcctccgcgggtgctcaaggctgaaggcgccggaccttcccccacggtggcacgcacatcatccggcaccatttccgtgccccgaagacgcccgcgcgggacctgggaccgccagtgaagaacccctcctgggctctttaacgagcagcagatgcgcatgctgcttctctccggcaggaaagccttctaagcccggcgtgctcgggcacccgagggtggaaccgcggcccctgcacacactcaccccaaagtctcaacgtcgaaccgaaggcgacacccacccaactcctccctctccgccccatagtccacccaacacttgcagcccctccagagaaaaagc

SEQ ID NO: 18563 - RNA, 1712 nt, Homo sapiens
  source 1..1712: mol_type = other RNA
tgagggagtgggtgggaggaaatagaatcacagcgggacacagggaggactcgaaagtattggttatgttctatttcctagtgtgtaattcttttattgttctttgtatcttacatatttattatagactgtatataagaaatgttttagttttaaaaaatcccacctctttggagcccaatgagagacacagcttctggcaggcactgatgaaatggaagtcacacctgccccccggaggcaaagcctttcactagttgggcctcctgcagatgttcctcagttctgtgctggtctccccagagctgcaggacagctggctgcacccagccctgggcatccttaggcttcctggctcctggcagattgctcctgtacggactgccacagagctctgatgttgccctgaccaaagccagtggccccctgcctctgaatcagctccaggaagaaagtgtcctcagtaaaaagggacttggtgaagacctgaagcagaaacttgcctttatcaccatctagcaggatcccctgtcgagcaagcagatgaggctcgtgccctgcagctcggatctgcctctcctttcctggctgctggtagtatgccccagggggagccaggaactggcctccagcagttgccaccccctcagtggcctccacaatgttaggcgtatacagccccacgtgctgcaggcctggccccttgtgccgggccaggaactgctccacctggtcctgtcgtgtcgtcgcccccggaagggactcagccagaacaagagtggggacaatgctgcccggctgggcctgcagggctgtaagcctcagtcccccaagcccaaaccctgctgtcatttcgaggcccagctcgggatcctcacctgggctcagcggcaagtggcaaaagcccaggcagtcgtggaaccagcgcaaaagtgtgggggagctgccgggggtgcaggccaaggtcaggtggtccacgcggctgacccacccggggccaggcgcagaggacacgggcctgaagccgggtaggaagggtccgcggtagccagcgcgctccagcaaggtcaggctgaggatgccggcaggcgagctgaccacggcgtaagtggcggcaccctgcgcgtcccgcacgcgaacgggagggacaggcacgctgcagcccagcgctgccagctcccgggttgcagcgccggcgtccgccacgtcgaagcacaggtttgtggcgctgggcacggcgtgacgcggatccaggccgtacagcggctctccagaccctgcgccctcgttcaccaaaaagaccgcgtcgccgctgcgcagggctagctgccgccagccgtccacctcccgcgaagccaggggctggaagccgaagaggcgctgcaggttccgggctaggggctgcccggcgggcacgtggaaggcgatgtggcacaaacgaagggcgggcgcggccatggcgctctggacggcgacctagacttgtccttctggggccgcttacttgtggttggggacttcggggctctcagtcctgggctgatcgtccggagttggggagtccggctcaccccgcagagcgcgttcctcgctttcttccggaaagaagtcacccgccgacccctgagagctcgcggttctccctgcagcgccaccccagccaggagcagcgtctggaccaccgggtctcagtgagccgagctgctggttgt

SEQ ID NO: 18564 - RNA, 2781 nt, Homo sapiens
  source 1..2781: mol_type = other RNA
tgagggagtgggtgggaggcaatttcacagggtctagcagataaatactggcatgttaacccacatttgcagtgtgaagaaacattattcactgaggttgaactaaaaaacagtattatttccccacacatttctcctgatcacttttctggaatggtcatttgtgcatcttgtgctgagagtgtgaatccaaagaatagactttctctgcgggtgactgaaaaaggaaagcgtggcaattgtcataggcacttccatctaaggagactgatagcattcttttctgctaaagaaataagaaaaaaacaagagaaatatgtaaaatttattgtttttaagctcactttgtcacatgcacacctgtgcatgcctatgtatgtgctcacccatgtgtgtatgaatgtgtttgtgcacactgcaaatgtgaactaagctgaggttggcctcctccagattacaacaggaggccttgagcattccccacttaccctggcaagtgagtgcatgaggatgcagggcaatgcctggcaaattgccgcgtgctcttttccctgatattagcctggctggtgtgccaggccctggggaagtgctgttacaggcactgaaggctacccctgtgaagcctctcaggctgatggatgggagtgagtctcaaagatctgtcaatcccgcctgtcagaagcctgccaaatgaaagatatgccaggctgactcaacaaaaagctcagcatcacccagcagaaatggctgctgaaggaagtgaagaaagatagaatggtggggggttgggggtggggagaggacaccaatagctctggttttacataggaggaacctgtttgacttgttaggtctgatttctgtgaacccgcagtttttcttggtgtcatcttaattatcttctgtgcaaagaaaaaaaggcagtgagtggcaataattaatttgcattgtcaattgatttttttttctttctaggaattcttctcactcaaaagccatattatataaccatctgtttttccccaaagatgaattctgttaggtttattcatttctgtctcttcagaagatatattaacattgccaatattgagcatctgtgtgtgtgagagcagagagagagattgagggagagatttggtggtttttccctttttaaacagttttgtgtcccttgacaccatttctcttgctttctggtttccaaactccagtggccattctcacttaggaacagatgctatgcaaaaatcagagcccaaacgtatcttactctgaggcttagatgggaaagagaacctttctcaaggtgaagatgaggaattcatgcaaatcaaaatttcagagaaagaggtctgcgttctattcttgctggcactatccttagaaggcacatgagttatccgctcagtttttacttcttttcttagaaaatggagagagtggtgcatcctccctttttggggggaaaaaagaggcaagaacaaaggaacacagtcattttctgcttttctacttttctgattttgtctttttgcttatttcattctctgataaaggaccagtattctcacctcctttatccctttattcaacagtttctgctaatttctgaataggcaaagaaagtatttgcacatgtacaatcgagggcagtgggcatgctcggcaagtacttggtccatggtgttctactccaagactgtcttctggagtaagctctgtccaaagttaggaggagggtggctgtttctgcccccttctttcctgaagtgatagagattggtctgtgactgctgctactgccaccgagcgaaattaagaaggggaaattaagaaggggaggatgtgagtaatagctccctccagacatctgcttgtgcttcggacccccacaaccctgggggaatggagagcagatctgaggtgatttgcctgaagccgttgcttggtaacctttccttttctcatggtttgacactcccctgggatattctattctctgagcacaaagtacaccaacaccagtagaaaaaaacctgtttgcttcctgtgtgttggtggcagaatgtcagagcctcctgcctagtaccccacagggctctgagcctggtcccttccgggttgtagtctctgatccccagattctaggatcttgctgaatggccagttccaagtgggtcagcacagcaagaggacatcaaattgtgaaacctactagttatggagctaggcagaactgaggttatgatgaggttcagagtttagacaatgaagctttgaggaaaattcccatagctgggaattcatagcagctttactgtacttcttaaacctcagacttagatgtgggaggagcacctggagttgatacaaagtagatgcagcagccagtggcactcaaattcagagtcagagctcccaacaaaattcagttaagaaatcacaacctagtcaattctcagcctgtaggctaaaatcaagtgtgagaaaatcgcagcccatagaccctagcccaaataaactggactctttccacaactatgctggccttttgcagtaagcctaagtgctttaaggatgtatctgttctggatctcactgttaggctgtggtcagacaggctggtgagctgggaaaagcctttgtgaggcccggaaactctttggtggctgggagcaacttgggaagggggaaatcccctctggccttatctgtccaagccctgctttcttctctcctctatcttccactcctttcttctctccacgagtgcct

SEQ ID NO: 18565 - RNA, 1087 nt, Homo sapiens
  source 1..1087: mol_type = other RNA
tgagggagtgggtgggagggaaaggctgggcagagcaggggaaggagtgaaagccaggcaggaaagtggaagaacaggagaagctcatgtaatggattaccctccacaggattatgttccttgattcctgagagttttttctcttgattttaccccctcagtctatcactgcaagagaaagaggtagaaaagacaaacagaccacaaaagacaagaacccagacatatagacagacgcacctgttgcatgtgcatgagccagagcctgggagagaagagagagcgtgcaagagagagctcagagcaggcaggcagcccaccccctgcagcagtgctgggcttcactggagcccctgcaggaagtccagcagccctgtatgccactcctctggtttgtccaggtaacaggggtgccccgcccccttcatgatcagcacccggtggttgggcagctgcttcaggtgctcaaagctggtctgacccatggggtcctggtctccatatacaatcagagctggagtcttcacactggcatagttggcagcattgattttgtcagtgcagatgggggccactggcacaaagcccgggagctgggagccaggggccgtgaggaagggcagggagtacatgccactcagtgatggactgatcacaaccggggggcccagctccaaggcatccaccacagccgccaggaagctgccaggggccagctccccaataggggcaggggctgctgcttccttggagtgccccagacctggcaggtcaatggccacagcccggtagccagcctgggccagcctgtgcagtgtacccaggttctgccaggtctcggaggagaagcgaataccatgcagcagcagtacagagaagcgagcctgcccactgccgggcagggcctctcggaagaagagggcctggccctgcacctggatggtgccctcgcgctgctccacgcttgctgccatgcctgctgctgctgtgctggtgaagggcctggggagctgcgtggactcgcgcagacgggaagcaggcgcgtgctggcggtgacctggggccggaggaggaacgctgggaagag

SEQ ID NO: 18566 - RNA, 1281 nt, Homo sapiens
  source 1..1281: mol_type = other RNA
tgagggagtgggtgggagggaaaggctgggcagagcaggggaaggagtgaaagccaggcaggaaagtggaagaacaggagaagctcatgtaatggattaccctccacaggattatgttccttgattcctgagagttttttctcttgattttaccccctcagtctatcactgcaagagaaagaggtagaaaagacaaacagaccacaaaagacaagaacccagacatatagacagacgcacctgttgcatgtgcatgagccagagcctgggagagaagagagagcgtgcaagagagagctcagagcaggcaggcagcccaccccctgcagcagtgctgggcttcactggagcccctgcaggaagtccagcagccctgtatgccactcctctggtttgtccaggtaacaggggtgccccgcccccttcatgatcagcacccggtggttgggcagctgcttcaggtgctcaaagctggtctgacccatggggtcctggtctccatatacaatcagagctggagtcttcacactggcatagttggcagcattgattttgtcagtgcagatgggggccactggcacaaagcccgggagctgggagccaggggccgtgaggaagggcagggagtacatgccactcagtgatggactgatcacaaccggggggcccagctccaaggcatccaccacagccgccaggaagctgccaggggccagctccccaataggggcaggggctgctgcttccttggagtgccccagacctggcaggtcaatggccacagcccggtagccagcctgggccagcctgtgcagtgtacccaggttctgccaggtctcggaggagaagcgaataccatgcagcagcagtacagagaagcgagcctgcccactgccgggcagggcctctcggaagaagagggcctggccctgcacctggatggtgccctcgcgctgctccacgcttgctgccatgcctgctgctgctgtgctggtgaagggcctgtggttcaaaaccacgatgatgaggggccacagaacaccctgcccagggtggcagtcccagaggagcagcaaggaagcctccaggaggtttccagaactttaagaacatgccttggggtcaggaggacataggtgttatttctgcctctgccatttactttagtgtgtaacctggggcctcagcttcttgatctggggagctgcgtggactcgcgcagacgggaagcaggcgcgtgctggcggtgacctggggccggaggaggaacgctgggaagag

SEQ ID NO: 18567 - RNA, 1429 nt, Homo sapiens
  source 1..1429: mol_type = other RNA
tgagggagtgggtgggagggaaaggctgggcagagcaggggaaggagtgaaagccaggcaggaaagtggaagaacaggagaagctcatgtaatggattaccctccacaggattatgttccttgattcctgagagttttttctcttgattttaccccctcagtctatcactgcaagagaaagaggtagaaaagacaaacagaccacaaaagacaagaacccagacatatagacagacgcacctgttgcatgtgcatgagccagagcctgggagagaagagagagcgtgcaagagagagctcagagcaggcaggcagcccaccccctgcagcagtgctgggcttcactggagcccctgcaggaagtccagcagccctgtatgccactcctctggtttgtccaggtaacaggggtgccccgcccccttcatgatcagcacccggtggttgggcagctgcttcaggtgctcaaagctggtctgacccatggggtcctggtctccatatacaatcagagctggagtcttcacactggcatagttggcagcattgattttgtcagtgcagatgggggccactggcacaaagcccgggagctgggagccaggggccgtgaggaagggcagggagtacatgccactcagtgatggactgatcacaaccggggggcccagctccaaggcatccaccacagccgccaggaagctgccaggggccagctccccaataggggcaggggctgctgcttccttggagtgccccagacctggggagctgcgtggactcgcgcagacgggaagcaggcgcgtgctggcggtgacctggggccggaggaggaacgctgggaagaggccgggccccatccagcgggggcggggactgggccgtgctccggggcgccctcttgtggccacaagctcgcagcgtccatagactccgctaaactcgttctcacagcggcgtcagtttcccaaagcctctcggtctcacatgccccaaacgcggtgctgagcacggtttcgaactcttcagcgacctgccccacatggacatggagcagtctgaggaggaaagttccttcgggatcgcatccttgctgctgtcttcctgctccccatcccccttatccccagcttgaactgcccagggcaacttgttggcctggcacggagttgaggcccgacaggtttgagtgcgaggctccgccagtgtccagccaagtggccttgatcgttttcccaatgcccccgagcctgtttcctgccagtagagcgggtcagatgttgccaacctctgcagagtagcaataagcagtaaacgccacgctctgcacagcctcccagtgctgggcctggtcgccacgcggagccttgggctgggacaggccagacgttggtaacacatcgccaaccagggcaggcgccatgagtag

SEQ ID NO: 18568 - RNA, 170 nt, Homo sapiens
  source 1..170: mol_type = other RNA
tgagggagtgggtgggagggccctggctgagcagctgcttcatcttcgtcatcatcatccagcacgatgatgctcagaaaccgtctctcgaggcgaccctcgccgcaattctcagaacctcgcatggttccctccgccttccttcccactcccaccgcaggccccactac

SEQ ID NO: 18569 - RNA, 236 nt, Homo sapiens
  source 1..236: mol_type = other RNA
tgagggagtgggtgggagggccctggctgagcagctgcttcatcttcgtcatcatcatccagcacgatgatgctgttagcggtggccataggggatcaaatcccccggagggaggaagtggtggggatttcagaattcctcagaaaccgtctctcgaggcgaccctcgccgcaattctcagaacctcgcatggttccctccgccttccttcccactcccaccgcaggccccactac

SEQ ID NO: 18570 - RNA, 239 nt, Homo sapiens
  source 1..239: mol_type = other RNA
tgagggagtgggtgggagggccctggctgagcagctgcttcatcttcgtcatcatcatccagcacgatgatgctgttagcggtggccataggggatcaaatcccccggagggaggaagtggtggggatttcagaattcctgctcagaaaccgtctctcgaggcgaccctcgccgcaattctcagaacctcgcatggttccctccgccttccttcccactcccaccgcaggccccactac

SEQ ID NO: 18571 - RNA, 926 nt, Homo sapiens
  source 1..926: mol_type = other RNA
tgaggggcagagagcgagactttctcaaaaaaaaaaaaaaaaacttaggttcttggatgttcgggaaagggggttattatctaggatccttgaagcacccccaagggcatcttctcaaagttggatgtgtgcattttcctgagaggaaagctttcccacattatacagcttctgaaagggttgcttgacccacagatgtgaagctgaggctgaaggagactgatgtggtttctcctcagtttctctgtgcggcaccaggtggcagcagaggtcagcaaggcaaacccgagcccagggatgcggggtgggggcagctacgtcctctcttgagctacagcagattcactctgttctgtttcattgttgcttagtttgcgttttgtttctccaactttgtacctcatcaggaaaagctttggatcacaattcccagtgctgaagaaaaggccaaactcttggttgtgttctttgatcagcgcctgtgacgcagcttcaggaggtcctgagaacgtgtgcacagtttagtcggcagaaacttagggaaacgtaagaccaccatcagtacgtaggagttgtgcattggtttggtccccatcccctgcataatgggtttctagctgcctcctctgcctgcccaaacaggacaggcaggaaaaactggcttggttctgagtaggcagtttcagggccttaaggagaaattcatcggccattaatcaggaccttccctccggggagttggcagcttcaggtgtggtctctggaaacaagccccacaaattattatcagagaacctctgtcttgggtggcagaggcagcctggttggggtgggcaccccggctacggaaaggagcagctccctccactttccttccggctgcatgtggagaggctcgagcggggcacagtccatgacgagatatt

SEQ ID NO: 18572 - RNA, 1327 nt, Homo sapiens
  source 1..1327: mol_type = other RNA
tgaggggcagagagcgagactttctcaaaaaaaaaaaaaaaaacttaggttcttggatgttcgggaaagggggttctttatctaggatccttgaagcacccccaagggcatcttctcaaagttggatgtgtgcattttcctgagaggaaagctttcccacattattcagcttctgaaagggttacttgacccacagatgtgaagctgaggctgaaggagactgatgtggtttctcctcagtttctctgtgtggcaccaggtggcagcagaggtcagcaaggcaaacccgagcccagggatgcggagtgggggcagctacgtcctctcttgagctacagcagattaactctgttctgtttcattgttgttgtttagtttgcttttttttctccaactttgtgcttcatcaggaaaagctttggatcacaattcccagtgctgaagaaaaggccaaactcttggttgtgttctttgatcagcgcctgtgacgcagcttcaggaggtcctgagaacgtgtgcacagtttagtcggcagaaacttagggaaacgtaagaccaccatcagtacgtaggagttgtgcattggtttggtcctgtcaaagggtgagcatttccggttcccctgctgtgctttgctgcgttgttctcccctgctgcaacgttctcactccacaatcctggggcaggtaggggaggcccagctgagtttggatcataatcccaggtcagctcctttctgcccactctttcagcgcaggcgtgtcctgctgtggaacacactctgggattcctgtgtgggtctgtacccatcctgtacccgtcaggacccccgggccctgactcttgatgttgttcttgctcctcttgttgatcttgttgttcccacagtgaggtccagtccagagagtatgcaagcacgaccacgtcaacaggccctgaagtcacaggttcacacagcacgttttctgctccatcacgtgtatggggcagggggcagcagagcagatcagactttgagctctcctcctggcttagcctggatcgtttgaaatggtcatccatcctttggccccaatacctaaactaaggtctatgaacaataagatgattttcttcagtgggacttttttgtttaatataatattagatatttcccctgatacagggctcaatctttttctttttaaagcaatatttctcaaagtacttttcacagaacttaagtttcattaagcacttcactaaaagaaaagtctgtgatctaataaatttggaaaatattgagaattagagccccctcttagatatgtactgtagctactcagct

SEQ ID NO: 18573 - RNA, 1407 nt, Homo sapiens
  source 1..1407: mol_type = other RNA
tgaggggcagagagcgagactttctcaaaaaaaaaaaaaaaaacttaggttcttggatgttcgggaaagggggttctttatctaggatccttgaagcacccccaagggcatcttctcaaagttggatgtgtgcattttcctgagaggaaagctttcccacattattcagcttctgaaagggttacttgacccacagatgtgaagctgaggctgaaggagactgatgtggtttctcctcagtttctctgtgtggcaccaggtggcagcagaggtcagcaaggcaaacccgagcccagggatgcggggtgggggcaggtacatcctctcttgagctacagcagattaactctgttctgtttcattgttgttgtttagtttgcttttttttctccaactttgtgcttcatcaggaaaagctttggatcacaattcccagtgctgaagaaaaggccaaactcttggttgtgttctttgattagtgcctgtgacgcagcttcaggaggtcctgagaacgtgtgcacagtttagtcggcagaaacttagggaaatgtaagaccaccatcagcacataggagttctgcattggtttggtctgcattggtttggtcttttcctggatacaggtcttgataggtctcttgatgtcatttcacttcagattcttctttagaaaacttcgacaatagcatttgctgtcttgtccaaattgttactaagaatcaagagagatatgatgtttgtctttctttgtatcagtgctcagctgagtctgcagtgcttcagaggcagctttcattttataaaaatctatgatttctccttccagttgttttttctcttcctcgagcttccttatctcctcctgttgaatcattttaagatgctcgaatttgtcctgcagtttgaccacataattgaaccttcgggtatcttgaattgcacttgagaagtctaaccgattaaaggtttctcccaaggtgcaatagccatgccttttgagtatttgtgtcatttctaaaatggtcctttttctttttttggatgcatattcatgctcttcattattgagtatttctccatcttcgctatttaagataatgctgtgactgatgttacaatggttattctctctttcaagtttctgactacaagattcacaattcttccagccatcttctgtcttaatccaactccatccaggagatctccagtcctgacccaaaaatggcatagttctcctagcgcgcctgcagcccccagtcttcacctgacgcgcccgcgtcccccagtgcccaacgggcgcgcctgccacctgggccggcacctgacggcgaccaggcgattattgccggaagtgggccaccgcctctcggcgcgcctcagggaagccccgcccctggccatgct

SEQ ID NO: 18574 - RNA, 1283 nt, Homo sapiens
  source 1..1283: mol_type = other RNA
tgaggggcagagagcgagactttctcaaaaaaaaaaaaaaaaacttaggttcttggatgttcgggaaagggggttctttatctaggatccttgaagcacccccaagggcatcttctcaaagttggatgtgtgcattttcctgagaggaaagctttcccacattattcagcttctgaaagggttacttgacccacagatgtgaagctgaggctgaaggagactgatgtggtttctcctcagtttctctgtgtggcaccaggtggcagcagaggtcagcaaggcaaacccgagcccagggatgcggggtgggggcaggtacatcctctcttgagctacagcagattaactctgttctgtttcattgttgttgtttagtttgcttttttttctccaactttgtgcttcatcaggaaaagctttggatcacaattcccagtgctgaagaaaaggccaaactcttggttgtgttctttgattagtgcctgtgacgcagcttcaggaggtcctgagaacgtgtgcacagtttagtcggcagaaacttagggaaatgtaagaccaccatcagcacataggagttctgcattggtttggtctgcattggtttggtcttttcctggatacaggtcttgataggtctcttgatgtcatttcacttcagattcttctttagaaaacttcgacaatagcatttgctgtcttgtccaaattgttacttcaagtttgctcttagcaagtaattgtttcagtatctatatcaaaaatggcttaagtctgcaacatgtttctgaatgattaacaaggtgatagtcagttcttcattgaatcctggatgctttatttttcttaataagaggaattcatatggatcagtttgagtatttgtgtcatttctaaaatggtcctttttctttttttggatgcatattcatgctcttcattattgagtatttctccatcttcgctatttaagataatgctgtgactgatgttacaatggttattctctctttcaagtttctgactacaagattcacaattcttccagccatcttctgtcttaatccaactccatccaggagatctccagtcctgacccaaaaatggcatagttctcctagcgcgcctgcagcccccagtcttcacctgacgcgcccgcgtcccccagtgcccaacgggcgcgcctgccacctgggccggcacctgacggcgaccaggcgattattgccggaagtgggccaccgcctctcggcgcgcctcagggaagccccgcccctggccatgct

SEQ ID NO: 18575 - RNA, 1179 nt, Homo sapiens
  source 1..1179: mol_type = other RNA
tgaggggcagagagcgagactttctcaaaaaaaaaaaaaaaaacttaggttcttggatgttcgggaaagggggttctttatctaggatccttgaagcacccccaagggcatcttctcaaagttggatgtgtgcattttcctgagaggaaagctttcccacattattcagcttctgaaagggttacttgacccacagatgtgaagctgaggctgaaggagactgatgtggtttctcctcagtttctctgtgtggcaccaggtggcagcagaggtcagcaaggcaaacccgagcccagggatgcggggtgggggcaggtacatcctctcttgagctacagcagattaactctgttctgtttcattgttgttgtttagtttgcttttttttctccaactttgtgcttcatcaggaaaagctttggatcacaattcccagtgctgaagaaaaggccaaactcttggttgtgttctttgattagtgcctgtgacgcagcttcaggaggtcctgagaacgtgtgcacagtttagtcggcagaaacttagggaaatgtaagaccaccatcagcacataggagttctgcattggtttggtctgcattggtttggtgatgtttgtctttctttgtatcagtgctcagctgagtctgcagtgcttcagaggcagctttcattttataaaaatctatgatttctccttccagttgttttttctcttcctcgagcttccttatctcctcctgttgaatcattttaagatgctcgaatttgtcctgcagtttgaccacataattgaaccttcgggtatcttgaattgcacttgagaagtctaaccgattaaaggtttctcccaaggtgcaatagccatgcctatgctgtgactgatgttacaatggttattctctctttcaagtttctgactacaagattcacaattcttccagccatcttctgtcttaatccaactccatccaggagatctccagtcctgacccaaaaatggcatagttctcctagcgcgcctgcagcccccagtcttcacctgacgcgcccgcgtcccccagtgcccaacgggcgcgcctgccacctgggccggcacctgacggcgaccaggcgattattgccggaagtgggccaccgcctctcggcgcgcctcagggaagccccgcccctggccatgct

SEQ ID NO: 18576 - RNA, 1332 nt, Homo sapiens
  source 1..1332: mol_type = other RNA
tgaggggcagagagcgagactttctcaaaaaaaaaaaaaaaaacttaggttcttggatgttcgggaaagggggttctttatctaggatccttgaagcacccccaagggcatcttctcaaagttggatgtgtgcattttcctgagaggaaagctttcccacattattcagcttctgaaagggttacttgacccacagatgtgaagctgaggctgaaggagactgatgtggtttctcctcagtttctctgtgtggcaccaggtggcagcagaggtcagcaaggcaaacccgagcccagggatgcggggtgggggcaggtacatcctctcttgagctacagcagattaactctgttctgtttcattgttgttgtttagtttgcttttttttctccaactttgtgcttcatcaggaaaagctttggatcacaattcccagtgctgaagaaaaggccaaactcttggttgtgttctttgattagtgcctgtgacgcagcttcaggaggtcctgagaacgtgtgcacagtttagtcggcagaaacttagggaaatgtaagaccaccatcagcacataggagttctgcattggtttggtctgcattggtttggtgatgtttgtctttctttgtatcagtgctcagctgagtctgcagtgcttcagaggcagctttcattttataaaaatctatgatttctccttccagttgttttttctcttcctcgagcttccttatctcctcctgttgaatcattttaagatgctcgaatttgtcctgcagtttgaccacataattgaaccttcgggtatcttgaattgcacttgagaagtctaaccgattaaaggtttctcccaaggtgcaatagccatgcctttcttttgtgctttctttatggacatagatccatttttcatgataaaaactttgagtatttgtgtcatttctaaaatggtcctttttctttttttggatgcatattcatgctcttcattattgagtatttctccatcttcgctatttaagataatgctgtgactgatgttacaatggttattctctctttcaagtttctgactacaagattcacaattcttccagccatcttctgtcttaatccaactccatccaggagatctccagtcctgacccaaaaatggcatagttctcctagcgcgcctgcagcccccagtcttcacctgacgcgcccgcgtcccccagtgcccaacgggcgcgcctgccacctgggccggcacctgacggcgaccaggcgattattgccggaagtgggccaccgcctctcggcgcgcctcagggaagccccgcccctggccatgct

SEQ ID NO: 18577 - RNA, 1986 nt, Homo sapiens
  source 1..1986: mol_type = other RNA
tgaggggcagagagcgagactttctcaaaaaaaaaaaaaaaacttaggttcttggatgttcgggaaagggggttattatctaggatccttgaagcgcccccaagggcatcttctcaaagttggatgtgtgcattttcctgagaggaaagctttcccacattatacagcttctgaaagggttgcttgacccacagatgtgaagctgaggctgaaggagactgatgtggtttctcctcagtttctctgtgcggcaccaggtggcagcagaggtcagcaaggcaaacccgagcccagggatgcggggtgggggcagctacgtcctctcttgagctacagcagattcactctgttctgtttcattgttgcttagtttgcgttttgtttctccaactttgtgcctcatcaggaaaagctttggatcacaattcccagtgctgaagaaaaggccaaactcttggttgtgttctttgatcagcgcctgtgacgcagcttcaggaggtcctgagaacgtgtgcacagtttagtcggcagaaacttagggaaacgtaagaccaccatcagtacgtaggagttgtgcattggtttggtccaggtcagctcctttctgcccactctttcagcgcaggcgtgtcctgctgtggaacacactctgggattcctgtgtgggtctgtacccgtcctgtacccgtcaggacccccgggccctgactcttgatgttgttcttgctcctcttgttgatcttgttgttcccacagtgaggtccagtccagagagtatgcaagcacgaccacgtcaacaggccctgaagtcacaggttcacacagcacgttttctgctccatcacgtgtatggggcagggggcagcagagcagatcagactttgagctctcctcctggcttagcctggatcgtttgaaatggtcatccatcctttggccccaatacctaaactaaggtctatgaacaataagatgattttcttcagtgggacttttttgtttaatataatattagatatttcccctgatacagggctcaatctttttctttttaaagcaatatttctcaaagtacttttcacagaacttaagtttcattaagcacttcactaaaagaaaagtctgtgatctaataaatttggaaaatattgagaattagagccccctcttagatatgtactgtagctactcagcttgttacagatgaagtaaacattgtaatattcacccagcttttgagtgatgtctattaacgtcacccaaatgagtattccatggaatgcactttgcaaaaacctattattcaagaaaattctggagcatgaaagctattaacgataaacccattcacaaaatcacaccaaatatctaaaatcatgtttaaaatctcctagaaatgggttgaattgcccacttcagagacaaagtgattcttttgtaataacgagttttgtttagtgagtacttattatctcattgaatcctgaggactacctcacaaggtaagtatagctcttttcattacacatgacaaacaaggctcagagaggttaagtaacttgctcaagatcacaaaactgcagagtgacaaaactagaattttgaatctaagctcaaagggtcaccaaaccaaatttgggtccacccacccagcctatcaaagtcaagcactgatatcggcattgctgagacagaagttgaggaatttattgcaggcagcaagcaaggagtatcaggcagctaatccttaaggcctaatctccctgatggcttatgtgtaagggtttttaaaggtgggaaggcagaggttgcaggcaaggtcatataatacatggaggctacatattggtttggccaaaaaaggcaaaatatctcaaagtgagggcccacaggataggtgaccattagatgaattcaaagattttctgatttgagaccaggtgcagtggttcacacctgtaatctcagcgctttgggaggccaagg

SEQ ID NO: 18578 - RNA, 800 nt, Homo sapiens
  source 1..800: mol_type = other RNA
tgaggggcagagagcgagactttctcaaaaaaaaaaaaaaaatcttaggttcttggatgttcgggaaagggggttattatctagaatccttgaagcgcccccaagggcatcttctcaaagttggatgtgtgcattttcctgagaggaaagctttcccacattattcagcttctgaaagggttacttgacccacagatgtgaagctgaggctgaaggagactgatgtggtttctcctcagtttctctgtgcggcaccaggtggcagcagaggtcagcaaggcaaacccgagcccggggatgcggagtgggggcagctacgtcctctcttgagctacagcagattcactctgttctgtttcattgttgttgtttagtttgcgttttttttctccaactttgtgcttcatcaggaaaagctttggatcacaattcccagtgctgaagaaaaggccaaactcttggttgtgttctttgattagtgcctgtgacgcagcttcaggaggtcctgagaacgtgtgcacagtttagtcggcagaaacttagggaaatgtaagaccaccatcagcacataggagttctgcattggtttggtctgcattggtttggtcttttcctggatacaggtcttgataggtctcttgatgtcatttcacttcagattcttctttagaaaacttggacaatagcatttgctgtcttgtccaaattgttaattcagcttaactatcattcagctcaggaagatgactcagggccttatccataccttcaagtttgctcttagcaagtaattgtttcag

SEQ ID NO: 18579 - RNA, 794 nt, Homo sapiens
  source 1..794: mol_type = other RNA
tgaggggcagagagcgagactttctcaaaaaaaaaaaaatcttaggttcttggatgttcgggaaagggggttattatctagaatccttgaagcgcccccaagggcatcttctcaaagttggatgtgtgcattttcctgagaggaaagctttcccacattatacagcttctgaaagggttgcttgacccacagatgtgaagctgaggctgaaggagactgatgtggtttctcctcagtttctctgtgtggcaccaggtggcagcagaggtcagcaaggcaaacccgagcccagggatgcggggtgggggcaggtacatcctctcttgagctacagcagattaactctgttctgtttcattgtggttgtttagtttgcgtttttttttctccaactttgtgcttcatcgggaaaagctttggatcacaattcccagtgctgaagaaaaggccaaactcttggttgtgttctttgattagtgcctgtgacgcagcttcaggaggtcctgagaacgtgtgcacagtttagtcggcagaaacttagggaaatgtaagaccaccatcagcacataggagttctgcattggtttggtctgcattggtttggtctgacaaagttgatttatcaagttgtaaatcttcacctgttgaattcataagttcatgtaaggagaaacatgtaaggatggcatgactcgccggcagccctgggattgtccacggtacccccatgatgaacagtaactccactgtgtaaacgcccatgaacctaagattacaagacttttccagtttag

SEQ ID NO: 18580 - RNA, 1740 nt, Homo sapiens
  source 1..1740: mol_type = other RNA
tgaggggcagagagcgagactttctcaaaaaaaaaaaaatcttaggttcttggatgttcgggaaagggggttattatctagaatccttgaagcgcccccaagggcatcttctcaaagttggatgtgtgcattttcctgagaggaaagctttcccacattatacagcttctgaaagggttgcttgacccacagatgtgaagctgaggctgaaggagactgatgtggtttctcctcagtttctctgtgtggcaccaggtggcagcagaggtcagcaaggcaaacccgagcccagggatgcggggtgggggcaggtacatcctctcttgagctacagcagattaactctgttctgtttcattgtggttgtttagtttgcgtttttttttctccaactttgtgcttcatcgggaaaagctttggatcacaattcccagtgctgaagaaaaggccaaactcttggttgtgttctttgattagtgcctgtgacgcagcttcaggaggtcctgagaacgtgtgcacagtttagtcggcagaaacttagggaaatgtaagaccaccatcagcacataggagttctgcattggtttggtctgcattggtttggtctgacaaagttgatttatcaagttgtaaatcttcacctgttgaattcataagttcatgtcatattttctttcagacaattcttcagtttgtttacgtagatcagcgatacgatgattccatttcttcggatccttgtaagagcagagcaggtgatggagagggtgggaggtgtagtgacagaagcaggaaactccagtcattcgagacgggcagcacaagctgcggagtgcaggccacctctacggccaggaaacggattctcccgcagagcctcggaagctaccgaccctgctcccaccttgactcagtaggacttactgtagaattctggccttcagacctgagcctggcagctctctccaactttggaagcccaggggcatggcccctgtccacagatgcacctggcatgaggcgtgcccagagggacagaggcagatgagtttcgtctcctccactggattgtgagggccagagttgaactccctcattttccgttccccagcattggcaggttctgggactggtggctgtggtggctcgttggtctttgtctcttagaaggtggggaataatcatcatcttgaaaaagaaaaaatggtcattactgaaggaaccatcttaggttacagccacctctgggtcaattcccaacattcaaaagctgagcagggctttaaagctatcttattaataattatttctgtattgcgaacttcagcatacttttttctagttacatttgaaatgttattcttttgggatgtgctcaagtgagtactgctttttcctctgccttgcttcattactttttagtttccttcatttgaatcatcattgtaagtctccccttctcctcaaataactttcaaattgctgccaagaactacgttctatcttaaggcttttgagaaaaaactttcaatgaagatagccgcctaaagttatacaaatatagaagaaacgggataaaataaagcttagattggaaaaaatatttaagattctacaaaattcacgcgtaaacaagggaagctgagtaattgtatgttcaaatacttttaacaagtgcaaaacatgtaggcttaaagaaatagagctggccaggcatggtggttcatgcctgtaattcca

SEQ ID NO: 18581 - RNA, 2126 nt, Homo sapiens
  source 1..2126: mol_type = other RNA
tgaggggcagagagcgagactttctcaaaaaaaaaaaaatcttaggttcttggatgttcgggaaagggggttattatctagaatccttgaagcgcccccaagggcatcttctcaaagttggatgtgtgcattttcctgagaggaaagctttcccacattatacagcttctgaaagggttgcttgacccacagatgtgaagctgaggctgaaggagactgatgtggtttctcctcagtttctctgtgtggcaccaggtggcagcagaggtcagcaaggcaaacccgagcccagggatgcggggtgggggcaggtacatcctctcttgagctacagcagattaactctgttctgtttcattgtggttgtttagtttgcgtttttttttctccaactttgtgcttcatcgggaaaagctttggatcacaattcccagtgctgaagaaaaggccaaactcttggttgtgttctttgattagtgcctgtgacgcagcttcaggaggtcctgagaacgtgtgcacagtttagtcggcagaaacttagggaaatgtaagaccaccatcagcacataggagttctgcattggtttggtctgcattggtttggtctgacaaagttgatttatcaagttgtaaatcttcacctgttgaattcataagttcatgtcttacaaggagaaacatgtaaggatggcatgactcgccggcagccctgggattgtccacggtacccccatgatgaacagtaactccactgtgtaaacgcccatgaacctaagattacaagacttttccagtttagacataccatattttctttcagacaattcttcagtttgtttacgtagatcagcgatacgatgattccatttcttcggatccttgtaagagcagagcaggtgatggagagggtgggaggtgtagtgacagaagcaggaaactccagtcattcgagacgggcagcacaagctgcggagtgcaggccacctctacggccaggaaacggattctcccgcagagcctcggaagctaccgaccctgctcccaccttgactcagtaggacttactgtagaattctggccttcagacctgagcctggcagctctctccaactttggaagcccaggggcatggcccctgtccacagatgcacctggcatgaggcgtgcccagagggacagaggcagatgagtttcgtctcctccactggattgtgagggccagagttgaactccctcattttccgttccccagcattggcaggttctgggactggtggctgtggtggctcgttggtctttgtctcttagaaggtggggaataatcatcatcttgaaaaagaaaaaatggtcattactgaaggaaccatcttaggttacagccacctctgggtcaattcccaacattcaaaagctgagcagggctttaaagctatcttattaataattatttctgtattgcgaacttcagcatacttttttctagttacatttgaaatgttattcttttgggatgtgctcaagtgagtactgctttttcctctgccttgcttcattactttttagtttccttcatttgaatcatcattgtaagtctccccttctcctcaaataactttcaaattgctgccaagaactacgttctatcttaaggcttttgagaaaaaactttcaatgaagatagccgcctaaagttatacaaatatagaagaaacgggataaaataaagcttagattggaaaaaatatttaagattctacaaaattcacgcgtaaacaagggaagctgagtaattgtatgttcaaatacttttaacaagtgcaaaacatgtaggcttaaagaaatagagctggccaggcatggtggttcatgcctgtaattccaacagtttgggaggccaaggcaggcagataacttgaggtcaggaattcgagaccagcctggccaacagagtgaaaccctctctctactaaaaatacaaaaattaggccaggagtgatggctcacgcctgtgatcccagcactttgagaggccgaggcgggtagatcacctgaggtcaggagtttgagaccagcctaaccaacatagggaaaccccgtctctactaaaactacaacattagccgggt

SEQ ID NO: 18582 - RNA, 629 nt, Homo sapiens
  source 1..629: mol_type = other RNA
tgaggggcagagagcgagactttctcaaaaaaaaaaaaatcttaggttcttggatgttcgggaaagggggttattatctagaatccttgaagcgcccccaagggcatcttctcaaagttggatgtgtgcattttcctgagaggaaagctttcccacattatacagcttctgaaagggttgcttgacccacagatgtgaagctgaggctgaaggagactgatgtggtttctcctcagtttctctgtgtggcaccaggtggcagcagaggtcagcaaggcaaacccgagcccagggatgcggggtgggggcaggtacatcctctcttgagctacagcagattaactctgttctgtttcattgtggttgtttagtttgcgtttttttttctccaactttgtgcttcatcgggaaaagctttggatcacaattcccagtgctgaagaaaaggccaaactcttggttgtgttctttgattagtgcctgtgacgcagcttcaggaggtcctgagaacgtgtgcacagtttagtcggcagaaacttagggaaatgtaagaccaccatcagcacataggagttctgcattggtttggtctgcattggtttggtcttcaagtttgctcttagcaagta

SEQ ID NO: 18583 - RNA, 804 nt, Homo sapiens
  source 1..804: mol_type = other RNA
tgaggggcagagagcgagactttctcaaaaaaaaaaaaatcttaggttcttggatgttcgggaaagggggttattatctagaatccttgaagcgcccccaagggcatcttctcaaagttggatgtgtgcattttcctgagaggaaagctttcccacattatacagcttctgaaagggttgcttgacccacagatgtgaagctgaggctgaaggagactgatgtggtttctcctcagtttctctgtgtggcaccaggtggcagcagaggtcagcaaggcaaacccgagcccagggatgcggggtgggggcaggtacatcctctcttgagctacagcagattaactctgttctgtttcattgtggttgtttagtttgcgtttttttttctccaactttgtgcttcatcgggaaaagctttggatcacaattcccagtgctgaagaaaaggccaaactcttggttgtgttctttgattagtgcctgtgacgcagcttcaggaggtcctgagaacgtgtgcacagtttagtcggcagaaacttagggaaatgtaagaccaccatcagcacataggagttctgcattggtttggtctgcattggtttggtcttttcctggatacaggtcttgataggtctcttgatgtcatttcacttcagattcttctttagaaaacttggacaatagcatttgctgtcttgtccaaattgttaattcagcttaactatcattcagctcaggaagatgactcagggccttatccataccttcaagtttgctcttagcaagtaattgtttcagtatcta

SEQ ID NO: 18584 - RNA, 762 nt, Homo sapiens
  source 1..762: mol_type = other RNA
tgaggggcagagagcgagactttctcaaaaaaaaaaaaatcttaggttcttggatgttcgggaaagggggttattatctagaatccttgaagcgcccccaagggcatcttctcaaagttggatgtgtgcattttcctgagaggaaagctttcccacattatacagcttctgaaagggttgcttgacccacagatgtgaagctgaggctgaaggagactgatgtggtttctcctcagtttctctgtgtggcaccaggtggcagcagaggtcagcaaggcaaacccgagcccagggatgcggggtgggggcaggtacatcctctcttgagctacagcagattaactctgttctgtttcattgtggttgtttagtttgcgtttttttttctccaactttgtgcttcatcgggaaaagctttggatcacaattcccagtgctgaagaaaaggccaaactcttggttgtgttctttgattagtgcctgtgacgcagcttcaggaggtcctgagaacgtgtgcacagtttagtcggcagaaacttagggaaatgtaagaccaccatcagcacataggagttctgcattggtttggtctgcattggtttggtcttttcctggatacaggtcttgataggtctcttgatgtcatttcacttcagattcttctttagaaaacttggacaatagcatttgctgtcttgtccaaattgttactcgaggcagctttgtaagcttctgagcacttcccaattccgggtgacttca

SEQ ID NO: 18585 - RNA, 66 nt, Homo sapiens
  source 1..66: mol_type = other RNA
tgaggggcagagagcgagacttttctattttccaaaagctcggtctgaggcccctcagtcttgctt

SEQ ID NO: 18586 - RNA, 73 nt, Homo sapiens
  source 1..73: mol_type = other RNA
tgaggggcctcagaccgagcttttggaaaatagaaaagtctcgctctctgcccctcagcctaacttcctttat

SEQ ID NO: 18587 - RNA, 292 nt, Homo sapiens
  source 1..292: mol_type = other RNA
tgagggtgtcagcaggtgacggattcttcgctgtgcagctggaatatcacagtatataatatggaccttggtgatgtaagttgtagctaaagtatatggatcagagggctgctttgctggaaacactttcagctcgctggcctctggtcatcttcattactactcccaagttgttttcactcaagcaatcttcttgccttggcctcccaaaatgttgggatcacaagtataatccaccatggcttgcctgaaacacattcttcaatgttctgtaattagttagtggaataga

SEQ ID NO: 18588 - RNA, 472 nt, Homo sapiens
  source 1..472: mol_type = other RNA
tgagggtgtcagcaggtgacggattcttcgctgtgcagctggaatatcacagtatataatatggaccttggtgatgtaagttgtagctaaagtatatggatcagagggctgctttgctggaaacactttcagctcgctggcctctggtcatcttcattactactcccaagttgttttcactgtaatcaactgtggtccaaaaatattaaatggaaaaatccggaagtaaacaattcatgatttaagttgcatgctgttctgagtagcgtgatgaaatcttgagctgtcctgcaccctctgtcttgcccgttccctagtccagagtatccatactgcagagctgcaggcacgcccagccattagttcttgacttaaggaaaggaaaattgcaggctgaggttgctaagatctatggtaagaatgaatcttctatcctggaaattctgttgcccaggctgaagcacaatggtac

SEQ ID NO: 18589 - RNA, 409 nt, Homo sapiens
  source 1..409: mol_type = other RNA
tgagggtgtcagcaggtgacggattcttcgctgtgcagctggaatatcacagtatataatatggaccttggtgatgtaagttgtagctaaagtatatggatcagagggctgctttgctggaaacactttcagctcgctggcctctggtcatcttcattactactcccaagttgttttcactgtaatcaactgtggtccaaaaatattaaatggaaaaatccggaagtaaacaattcatgatttaagttgcatgctgttctgagtagcgtgatgaaatcttgagctgtcctgcaccctctgtcttgcccgttccctagtccagagtatccatactgcagagctgcaggcacgcccagccattagttcttgatctgttgcccaggctgaagcacaatggtacaatcgcagc

SEQ ID NO: 18590 - RNA, 664 nt, Homo sapiens
  source 1..664: mol_type = other RNA
tgaggtaggaggttgtatagttgaggaggacacccaaggagatcactatacggcctcctagctttccccaggctgcgccctgcacgggacggggcccggcggggacccccagccccactcagggacccttagccccactgggctgccccagggaccctgggaggaagagccgggctcttttctgtccttgtccctgcatcccctccttcccctgaaatctgttttccttccctgtctgtctccatctctgctgtgtctctgtggcttctgtgtctctttcacagtggatcctctgactccctcttattctggctttctaggtctctgcccctcccgatatctctctgtgtctctatttctgtcgtttttggtctttctgtctctggctctcagaatgtctctgtgcctatctccatctctgacccccaccccagggtctaccgggccaccgcacaccatgttgccagtctctaggtccctgagaccctttaacctgtgaggacatccagggtcacaggtgaggttcttgggagcctggcgtctggcccaaccacacacctggggaattgctggcctgacttctgacccctgactcctcatacccttcctccagagcatgacatttgaccaccaactgaaacctgacctctgaccccagaccact

SEQ ID NO: 18591 - RNA, 71 nt, Homo sapiens
  source 1..71: mol_type = other RNA
tgaggtagtagattgtatagttatcccatagcagggcagagccccaaactatacaacctactacctcaccc

SEQ ID NO: 18592 - RNA, 3457 nt, Homo sapiens
  source 1..3457: mol_type = other RNA
tgaggtagtagattgtatagttatcccatagcagggcagagccccaaactatacaacctactacctcaccccaaagggcagtcggtcttggtgccgatgggactccgtggcttccagaggcacctcctggggacgcgggaggaaagagggctgaggagaacaggggctcgaggctcggcaggccacacgcaccaagggcacagggattctggcgggcaggcgcggtgggcgcagggggctgggacgccgaaaccctgggagtggggacattgtggccagcaccagcagggacgggagcctgcaggaaaccaccaaccagagagggacgaggaagagagaaaggaggagggagggaaagccctggcggcattttgcgacgctgtcacaggcagccggctccctctcatctggacaggagtggccataatgtccccaaggaactctgcactggagaccctaggaggagggctgtcatctgtcgaaggccagcaagacacaggcatgcgagtgcccaccctgctcggccccctccctccccgcacagcgccaccagaagcagcactcgtggcccccaggctggctgagtagcggcttcacgggcgtgccgtctcctcccactgggcaggcaggcatccctccccaggggccctggttctggccctgctgtgcaggctggcctgagctgaccgcactgcaggaggtggcgggaaggttctttccttccttgagggaagtggcctctaggggagagcagctgggggggtagtcacagaccctcaggtccacccagggtccagtgcctgtccctgcgggtgctggcacactcagtgccctagcttgggacgcacagggctgggacagagtgtagcatgaggatgacactgagagggcctcggggctcccctagcaggggaacgtggcgagagacgggcctccctaagccccgcctatcctgggcctggtgcagggtcagcctcaacaaatgctaattgtggctaccaccttcctggggaaaagctgagggggcagatacgactgtcaacccctcttaaacaggtgaggagaccgaggcccagagaggcaacgtgacctggatgtcacacagccaagggggcagcagagtgaggtccaaatgtcctgctccctgccaagcttttttttttttttttttttttttttttgagatggagtctcactctgtcccccaggctggagtgcagtggcgcgatctcggctcactgcaagctccgcctcctgggttcacgccattctcctgcctcagcctcccgagtagctgggactacaggcgcccgccactacgcccggctgattttttgtatttttagtagacagggggtttcaccgtgttagccaggatggtgttgatctcctgacctcgtgatccgcccgcctcagcctcccaaagtgctgggattacaggcatgagccactgcgcccggcctgcttcctgccaagttaaacggcatgctagctctcagctccccatgcccaagtggacttgaaaggtctaccccagccctccttccacagcccatcctgagcaggctgcctactccaggcaggccccaggctgggctggaccatttaatcctcacagccctggtaaggctgagatcacggatcccacttcatagtggagaaactgaggctcagggggtgctgaatctctagctctaggtgtctttgctctcagaagttggtcggggagggggtctgcttgctctctgggcacgtgtcctactccctcccgaggggcactggagcaaatcccaggtccttagccagcaaggagaccgctgaggctcacacctggtgccgcccacccagaactggagactgagatgctgactcacccaggagtggggaccaggagggccccgatgcagcccgaccctcctctgtcccagcatcatctcgcctggggtcgcgaagaccccgtgttccctcaaggcctcagaacaaaagcggtatgagagggtctgggggtcctgctcccctgctccaattctgggtcccctggctggtgggcaggaccaagatgtccctaaggactgtccgggcagagccagccagggtggggtgagggctgaagggacagtggctgagggtctccttggaccctcccagctgtggtgagtggccggagggggaagatcaaggccatcccagctcctctgagctgaggctgactcaggctgtcgcacacctcatgatcagctcccagtcaggtggtccaccctgagtgtccctgcgtctgcccccatctgcacccccgggaggtgccttgggggaggctgtggggtgggttgcaccctaagcacgcactctgggctcctgacttaatctctgagacccccaccccctcaggctggactggccacctgggctggctgggtcccctcacacctactgggttctgactcatggtcccagcaggctaaaaagggggtggggcaggacagcccagtgggcggagctgtgagaatccaggccggcctctgggctatgctctgggcaggtctcatgccctcgtgagccgtggtctccccactgaggcaaggggtcagctgccagggcccccgtcatcagccatcggagctggagtgcaggtggggaccaccatactgattccaatggccccagcctggcccccacaggtcccccaggccaggacttcagcctcctagagcctacagtgctcaccatggggggacccagcccacaggtcgggctctataacgtgtggcagagacagaatgggagacaggcccctagtccaccctggtcgtcaccacaagtgccctccccctgggcccccagccccacctgggagaagcagatgtgactcagtttccctcattcggcctttctcgttctgggctagacttacccaggtggcatcttgagtcatcctgggcgatggcaggtggcctcggggcatgagggctgcactccaggatgcccggtggctaggtgacaggagaggccagcgcaggagcttctgtccccagggagtgctcgaggcaggctgggccctccagagccaggatggcaggaggcccagctcactgtgaggaaggccagccccaggcaggggctccaggtcagcgccacttcttgacctgagggtggacacagtcccttgagcttcaggcatcacctggggaggtggccaagggtggaagacctgggccgttaggtcccggaggatcttccctagcccacgatgggctcctgatgtctcgggtggtgctctgggacggggccacatttatctcaagctgaaggcgccgtctccacgccgcccaggcttccaaatgcggccacacggactttgaagggcgtccgctgcagggtcacaggcgccagtgtctgctcgtctggacctcgaagcaccaggcccaggaggagtcctcctctcatcgagttgaaagaa

SEQ ID NO: 18593 - RNA, 3608 nt, Homo sapiens
  source 1..3608: mol_type = other RNA
tgaggtagtagattgtatagttatcccatagcagggcagagccccaaactatacaacctactacctcaccccaaagggcagtcggtcttggtgccgatgggactccgtggcttccagaggcacctcctggggacgcgggaggaaagagggctgaggagaacaggggctcgaggctcggcaggccacacgcaccaagggcacagggattctggcgggcaggcgcggtgggcgcagggggctgggacgccgaaaccctgggagtggggacattgtggccagcaccagcagggacgggagcctgcaggaaaccaccaaccagagagggacgaggaagagagaaaggaggagggagggaaagccctggcggcattttgcgacgctgtcacaggcagccggctccctctcatctggacaggagtggccataatgtccccaaggaactctgcactggagaccctaggaggagggctgtcatctgtcgaaggccagcaagacacaggcatgcgagtgcccaccctgctcggccccctccctccccgcacagcgccaccagaagcagcactcgtggcccccaggctggctgagtagcggcttcacgggcgtgccgtctcctcccactgggcaggcaggcatccctccccaggggccctggttctggccctgctgtgcaggctggcctgagctgaccgcactgcaggaggtggcgggaaggttctttccttccttgagggaagtggcctctaggggagagcagctgggggggtagtcacagaccctcaggtccacccagggtccagtgcctgtccctgcgggtgctggcacactcagtgccctagcttgggacgcacagggctgggacagagtgtagcatgaggatgacactgagagggcctcggggctcccctagcaggggaacgtggcgagagacgggcctccctaagccccgcctatcctgggcctggtgcagggtcagcctcaacaaatgctaattgtggctaccaccttcctggggaaaagctgagggggcagatacgactgtcaacccctcttaaacaggtgaggagaccgaggcccagagaggcaacgtgacctggatgtcacacagccaagggggcagcagagtgaggtccaaatgtcctgctccctgccaagcttttttttttttttttttttttttttttgagatggagtctcactctgtcccccaggctggagtgcagtggcgcgatctcggctcactgcaagctccgcctcctgggttcacgccattctcctgcctcagcctcccgagtagctgggactacaggcgcccgccactacgcccggctgattttttgtatttttagtagacagggggtttcaccgtgttagccaggatggtgttgatctcctgacctcgtgatccgcccgcctcagcctcccaaagtgctgggattacaggcatgagccactgcgcccggcctgcttcctgccaagttaaacggcatgctagctctcagctccccatgcccaagtggacttgaaaggtctaccccagccctccttccacagcccatcctgagcaggctgcctactccaggcaggccccaggctgggctggaccatttaatcctcacagccctggtaaggctgagatcacggatcccacttcatagtggagaaactgaggctcagggggtgctgaatctctagctctaggtgtctttgctctcagaagttggtcggggagggggtctgcttgctctctgggcacgtgtcctactccctcccgaggggcactggagcaaatcccaggtccttagccagcaaggagaccgctgaggctcacacctggtgccgcccacccagaactggagactgagatgctgactcacccaggagtggggaccaggagggccccgatgcagcccgaccctcctctgtcccagcatcatctcgcctggggtcgcgaagaccccgtgttccctcaaggcctcagaacaaaagcggtatgagagggtctgggggtcctgctcccctgctccaattctgggtcccctggctggtgggcaggaccaagatgtccctaaggactgtccgggcagagccagccagggtggggtgagggctgaagggacagtggctgagggtctccttggaccctcccagctgtggtgagtggccggagggggaagatcaaggccatcccagctcctctgagctgaggctgactcaggctgtcgcacacctcatgatcagctcccagtcaggtggtccaccctgagtgtccctgcgtctgcccccatctgcacccccgggaggtgccttgggggaggctgtggggtgggttgcaccctaagcacgcactctgggctcctgacttaatctctgagacccccaccccctcaggctggactggccacctgggctggctgggtcccctcacacctactgggttctgactcatggtcccagcaggctaaaaagggggtggggcaggacagcccagtgggcggagctgtgagaatccaggccggcctctgggctatgctctgggcaggtctcatgccctcgtgagccgtggtctccccactgaggcaaggggtcagctgccagggcccccgtcatcagccatcggagctggagtgcaggtggggaccaccatactgattccaatggccccagcctggcccccacaggtcccccaggccaggacttcagcctcctagagcctacagtgctcaccatggggggacccagcccacaggtcgggctctataacgtgtggcagagacagaatgggagacaggcccctagtccaccctggtcgtcaccacaagtgccctccccctgggcccccagccccacctgggagaagcagatgtgactcagtttccctcattcggcctttctcgttctgggctagacttacccaggtggcatcttgagtcatcctgggcgatggcaggtggcctcggggcatgagggctgcactccaggatgcccggtggctaggtgacaggagaggccagcgcaggagcttctgtccccagggagtgctcgaggcaggctgggccctgcagacaggcggtgcacacaacagagcccagggccagagagtgagtcttcagggtgtggaggtgaggctgagcctcttccactcagacgccctccagagccaggatggcaggaggcccagctcactgtgaggaaggccagccccaggcaggggctccaggtcagcgccacttcttgacctgaggactcagcccaggcctctgatggggaccgccgatccagagccacgggcagggcctgagggtggacacagtcccttgagcttcaggcatcacctggggaggtggccaagggtggaagacctgggccgttaggtcccggaggatcttccctagcccacgatgggctcctgatgtctcgggtggtgctctgggacggggccacatttatctcaagctgaaggcgccgtctccacgccgcccaggcttccaaatgcggccacacggactttgaagggcgtccgctgcagggtcacaggcgccagtgtctgctcgtctggacctcgaagcaccaggcccaggaggagtcctcctctcatcgagttgaaagaa

SEQ ID NO: 18594 - RNA, 76 nt, Homo sapiens
  source 1..76: mol_type = other RNA
tgaggtagtagattgtatagttatctcccagtggtgggtgtgaccctaaaactatacaacctactacctcatccca

SEQ ID NO: 18595 - RNA, 292 nt, Homo sapiens
  source 1..292: mol_type = other RNA
tgaggtagtagattgtatagttatctcccagtggtgggtgtgaccctaaaactatacaacctactacctcatcccacagtgaagagaacatccagggtgaatggtgaaaaggaatcacagttgagcaccacaggaaggctttttttcctcctcggtaatcctggtttcctcgcgctcgcggagagggccgtcgcggccgtgggaatgccccggccctcgcgcccgtcgctgccgggagagcaccgcgccaggacccggatggaggcgcgggcgggcgccgccgcggcggcct

SEQ ID NO: 18596 - RNA, 79 nt, Homo sapiens
  source 1..79: mol_type = other RNA
tgaggtagtaggttgtatagttatcttccgaggggcaacatcactgccctgaaaccacacaacctactacctcaccccg

SEQ ID NO: 18597 - RNA, 4402 nt, Homo sapiens
  source 1..4402: mol_type = other RNA
tgaggtagtaggttgtatagttatcttccgaggggcaacatcactgccctgaaaccacacaacctactacctcaccccgccaggcccggccttgcactgcgggagggcccgccgccccccgcccagcaccagcccctgcctggcggtcctcagtcaccagagcaggagggctgggcaggcgcagggcaggagggacaggggagatggcaccccaggaaggggcagctgctgctggctggtcttgggaagtccctggctctctgggcctcagtttccccaggtacagaggagccactgtctgccttcagattgtgccatgtgggacccagtgtatgcagagctgttcctctcacttcctgctcaggaaaggtgccttggcctcccttcctccacaggcagaggccctgccactgagctggccaggctggggcacgtgctgggaacctggggtgatgggcaacgccaatactcgcagccctgtgacctccaaacgtctcggccacccctggccccacggtgccttctcctggtgctcagtggagggtacggctcagggccacccatgagcctgggcctgatggcggggggagtgttggggagtgttgggagacagaggtcagacaaacagctgcgtggatcgcctctctcagtgcggctggggcagagggtggggtcggctcagctctcctctgccctcgatgctccacactgcatctccttccatcctcatttgcctccattttacagaggaggaaactgagacccagagagatcaggggcctgtccaaggtcacacagcaagtggcacctaggcctgtcagacttctcagtgtaggcggcccctgcccccgactgctgccaaggctgcccccaaacctggccctgcccgctcccagccagggttccagacgctctgtccaccgcagatattacagccacttcaggaaagacagtagattgtatagttatcccatagcagggcagagccccaaactatacaacctactacctcaccccaaagggcagtcggtcttggtgccgatgggactccgtggcttccagaggcacctcctggggacgcgggaggaaagagggctgaggagaacaggggctcgaggctcggcaggccacacgcaccaagggcacagggattctggcgggcaggcgcggtgggcgcagggggctgggacgccgaaaccctgggagtggggacattgtggccagcaccagcagggacgggagcctgcaggaaaccaccaaccagagagggacgaggaagagagaaaggaggagggagggaaagccctggcggcattttgcgacgctgtcacaggcagccggctccctctcatctggacaggagtggccataatgtccccaaggaactctgcactggagaccctaggaggagggctgtcatctgtcgaaggccagcaagacacaggcatgcgagtgcccaccctgctcggccccctccctccccgcacagcgccaccagaagcagcactcgtggcccccaggctggctgagtagcggcttcacgggcgtgccgtctcctcccactgggcaggcaggcatccctccccaggggccctggttctggccctgctgtgcaggctggcctgagctgaccgcactgcaggaggtggcgggaaggttctttccttccttgagggaagtggcctctaggggagagcagctgggggggtagtcacagaccctcaggtccacccagggtccagtgcctgtccctgcgggtgctggcacactcagtgccctagcttgggacgcacagggctgggacagagtgtagcatgaggatgacactgagagggcctcggggctcccctagcaggggaacgtggcgagagacgggcctccctaagccccgcctatcctgggcctggtgcagggtcagcctcaacaaatgctaattgtggctaccaccttcctggggaaaagctgagggggcagatacgactgtcaacccctcttaaacaggtgaggagaccgaggcccagagaggcaacgtgacctggatgtcacacagccaagggggcagcagagtgaggtccaaatgtcctgctccctgccaagcttttttttttttttttttttttttttttgagatggagtctcactctgtcccccaggctggagtgcagtggcgcgatctcggctcactgcaagctccgcctcctgggttcacgccattctcctgcctcagcctcccgagtagctgggactacaggcgcccgccactacgcccggctgattttttgtatttttagtagacagggggtttcaccgtgttagccaggatggtgttgatctcctgacctcgtgatccgcccgcctcagcctcccaaagtgctgggattacaggcatgagccactgcgcccggcctgcttcctgccaagttaaacggcatgctagctctcagctccccatgcccaagtggacttgaaaggtctaccccagccctccttccacagcccatcctgagcaggctgcctactccaggcaggccccaggctgggctggaccatttaatcctcacagccctggtaaggctgagatcacggatcccacttcatagtggagaaactgaggctcagggggtgctgaatctctagctctaggtgtctttgctctcagaagttggtcggggagggggtctgcttgctctctgggcacgtgtcctactccctcccgaggggcactggagcaaatcccaggtccttagccagcaaggagaccgctgaggctcacacctggtgccgcccacccagaactggagactgagatgctgactcacccaggagtggggaccaggagggccccgatgcagcccgaccctcctctgtcccagcatcatctcgcctggggtcgcgaagaccccgtgttccctcaaggcctcagaacaaaagcggtatgagagggtctgggggtcctgctcccctgctccaattctgggtcccctggctggtgggcaggaccaagatgtccctaaggactgtccgggcagagccagccagggtggggtgagggctgaagggacagtggctgagggtctccttggaccctcccagctgtggtgagtggccggagggggaagatcaaggccatcccagctcctctgagctgaggctgactcaggctgtcgcacacctcatgatcagctcccagtcaggtggtccaccctgagtgtccctgcgtctgcccccatctgcacccccgggaggtgccttgggggaggctgtggggtgggttgcaccctaagcacgcactctgggctcctgacttaatctctgagacccccaccccctcaggctggactggccacctgggctggctgggtcccctcacacctactgggttctgactcatggtcccagcaggctaaaaagggggtggggcaggacagcccagtgggcggagctgtgagaatccaggccggcctctgggctatgctctgggcaggtctcatgccctcgtgagccgtggtctccccactgaggcaaggggtcagctgccagggcccccgtcatcagccatcggagctggagtgcaggtggggaccaccatactgattccaatggccccagcctggcccccacaggtcccccaggccaggacttcagcctcctagagcctacagtgctcaccatggggggacccagcccacaggtcgggctctataacgtgtggcagagacagaatgggagacaggcccctagtccaccctggtcgtcaccacaagtgccctccccctgggcccccagccccacctgggagaagcagatgtgactcagtttccctcattcggcctttctcgttctgggctagacttacccaggtggcatcttgagtcatcctgggcgatggcaggtggcctcggggcatgagggctgcactccaggatgcccggtggctaggtgacaggagaggccagcgcaggagcttctgtccccagggagtgctcgaggcaggctgggccctccagagccaggatggcaggaggcccagctcactgtgaggaaggccagccccaggcaggggctccaggtcagcgccacttcttgacctgagggtggacacagtcccttgagcttcaggcatcacctggggaggtggccaagggtggaagacctgggccgttaggtcccggaggatcttccctagcccacgatgggctcctgatgtctcgggtggtgctctgggacggggccacatttatctcaagctgaaggcgccgtctccacgccgcccaggcttccaaatgcggccacacggactttgaagggcgtccgctgcagggtcacaggcgccagtgtctgctcgtctggacctcgaagcaccaggcccaggaggagtcctcctctcatcgagttgaaagaa

SEQ ID NO: 18598 - RNA, 4553 nt, Homo sapiens
  source 1..4553: mol_type = other RNA
tgaggtagtaggttgtatagttatcttccgaggggcaacatcactgccctgaaaccacacaacctactacctcaccccgccaggcccggccttgcactgcgggagggcccgccgccccccgcccagcaccagcccctgcctggcggtcctcagtcaccagagcaggagggctgggcaggcgcagggcaggagggacaggggagatggcaccccaggaaggggcagctgctgctggctggtcttgggaagtccctggctctctgggcctcagtttccccaggtacagaggagccactgtctgccttcagattgtgccatgtgggacccagtgtatgcagagctgttcctctcacttcctgctcaggaaaggtgccttggcctcccttcctccacaggcagaggccctgccactgagctggccaggctggggcacgtgctgggaacctggggtgatgggcaacgccaatactcgcagccctgtgacctccaaacgtctcggccacccctggccccacggtgccttctcctggtgctcagtggagggtacggctcagggccacccatgagcctgggcctgatggcggggggagtgttggggagtgttgggagacagaggtcagacaaacagctgcgtggatcgcctctctcagtgcggctggggcagagggtggggtcggctcagctctcctctgccctcgatgctccacactgcatctccttccatcctcatttgcctccattttacagaggaggaaactgagacccagagagatcaggggcctgtccaaggtcacacagcaagtggcacctaggcctgtcagacttctcagtgtaggcggcccctgcccccgactgctgccaaggctgcccccaaacctggccctgcccgctcccagccagggttccagacgctctgtccaccgcagatattacagccacttcaggaaagacagtagattgtatagttatcccatagcagggcagagccccaaactatacaacctactacctcaccccaaagggcagtcggtcttggtgccgatgggactccgtggcttccagaggcacctcctggggacgcgggaggaaagagggctgaggagaacaggggctcgaggctcggcaggccacacgcaccaagggcacagggattctggcgggcaggcgcggtgggcgcagggggctgggacgccgaaaccctgggagtggggacattgtggccagcaccagcagggacgggagcctgcaggaaaccaccaaccagagagggacgaggaagagagaaaggaggagggagggaaagccctggcggcattttgcgacgctgtcacaggcagccggctccctctcatctggacaggagtggccataatgtccccaaggaactctgcactggagaccctaggaggagggctgtcatctgtcgaaggccagcaagacacaggcatgcgagtgcccaccctgctcggccccctccctccccgcacagcgccaccagaagcagcactcgtggcccccaggctggctgagtagcggcttcacgggcgtgccgtctcctcccactgggcaggcaggcatccctccccaggggccctggttctggccctgctgtgcaggctggcctgagctgaccgcactgcaggaggtggcgggaaggttctttccttccttgagggaagtggcctctaggggagagcagctgggggggtagtcacagaccctcaggtccacccagggtccagtgcctgtccctgcgggtgctggcacactcagtgccctagcttgggacgcacagggctgggacagagtgtagcatgaggatgacactgagagggcctcggggctcccctagcaggggaacgtggcgagagacgggcctccctaagccccgcctatcctgggcctggtgcagggtcagcctcaacaaatgctaattgtggctaccaccttcctggggaaaagctgagggggcagatacgactgtcaacccctcttaaacaggtgaggagaccgaggcccagagaggcaacgtgacctggatgtcacacagccaagggggcagcagagtgaggtccaaatgtcctgctccctgccaagcttttttttttttttttttttttttttttgagatggagtctcactctgtcccccaggctggagtgcagtggcgcgatctcggctcactgcaagctccgcctcctgggttcacgccattctcctgcctcagcctcccgagtagctgggactacaggcgcccgccactacgcccggctgattttttgtatttttagtagacagggggtttcaccgtgttagccaggatggtgttgatctcctgacctcgtgatccgcccgcctcagcctcccaaagtgctgggattacaggcatgagccactgcgcccggcctgcttcctgccaagttaaacggcatgctagctctcagctccccatgcccaagtggacttgaaaggtctaccccagccctccttccacagcccatcctgagcaggctgcctactccaggcaggccccaggctgggctggaccatttaatcctcacagccctggtaaggctgagatcacggatcccacttcatagtggagaaactgaggctcagggggtgctgaatctctagctctaggtgtctttgctctcagaagttggtcggggagggggtctgcttgctctctgggcacgtgtcctactccctcccgaggggcactggagcaaatcccaggtccttagccagcaaggagaccgctgaggctcacacctggtgccgcccacccagaactggagactgagatgctgactcacccaggagtggggaccaggagggccccgatgcagcccgaccctcctctgtcccagcatcatctcgcctggggtcgcgaagaccccgtgttccctcaaggcctcagaacaaaagcggtatgagagggtctgggggtcctgctcccctgctccaattctgggtcccctggctggtgggcaggaccaagatgtccctaaggactgtccgggcagagccagccagggtggggtgagggctgaagggacagtggctgagggtctccttggaccctcccagctgtggtgagtggccggagggggaagatcaaggccatcccagctcctctgagctgaggctgactcaggctgtcgcacacctcatgatcagctcccagtcaggtggtccaccctgagtgtccctgcgtctgcccccatctgcacccccgggaggtgccttgggggaggctgtggggtgggttgcaccctaagcacgcactctgggctcctgacttaatctctgagacccccaccccctcaggctggactggccacctgggctggctgggtcccctcacacctactgggttctgactcatggtcccagcaggctaaaaagggggtggggcaggacagcccagtgggcggagctgtgagaatccaggccggcctctgggctatgctctgggcaggtctcatgccctcgtgagccgtggtctccccactgaggcaaggggtcagctgccagggcccccgtcatcagccatcggagctggagtgcaggtggggaccaccatactgattccaatggccccagcctggcccccacaggtcccccaggccaggacttcagcctcctagagcctacagtgctcaccatggggggacccagcccacaggtcgggctctataacgtgtggcagagacagaatgggagacaggcccctagtccaccctggtcgtcaccacaagtgccctccccctgggcccccagccccacctgggagaagcagatgtgactcagtttccctcattcggcctttctcgttctgggctagacttacccaggtggcatcttgagtcatcctgggcgatggcaggtggcctcggggcatgagggctgcactccaggatgcccggtggctaggtgacaggagaggccagcgcaggagcttctgtccccagggagtgctcgaggcaggctgggccctgcagacaggcggtgcacacaacagagcccagggccagagagtgagtcttcagggtgtggaggtgaggctgagcctcttccactcagacgccctccagagccaggatggcaggaggcccagctcactgtgaggaaggccagccccaggcaggggctccaggtcagcgccacttcttgacctgaggactcagcccaggcctctgatggggaccgccgatccagagccacgggcagggcctgagggtggacacagtcccttgagcttcaggcatcacctggggaggtggccaagggtggaagacctgggccgttaggtcccggaggatcttccctagcccacgatgggctcctgatgtctcgggtggtgctctgggacggggccacatttatctcaagctgaaggcgccgtctccacgccgcccaggcttccaaatgcggccacacggactttgaagggcgtccgctgcagggtcacaggcgccagtgtctgctcgtctggacctcgaagcaccaggcccaggaggagtcctcctctcatcgagttgaaagaa

SEQ ID NO: 18599 - RNA, 3395 nt, Homo sapiens
  source 1..3395: mol_type = other RNA
tgaggtagtagtttcttggatggtgctgcaaaattgaaatggccttggtgttcctttccactcttgggtagagccgggtagagggctgctagagtccaaggaccttccacaactcggacaggaggtttcatggctatgtgcaaatctatctatctatctatcttcctcattcttacttccactctgagtatctgtgcgagtgctggaggtttcaaacaatttttctttttcagtctctctccgccagtgaaaacaaaatatggcaacaataaaaagcacagaaatgatatctgcaaggagccacatgaacacatagaactttggtgtcagatgttgctcgattttagaggcaaggatcacgcttactacttggcggacaaatgtgtgtctgagaggatgttttggtggagggcgatgaagatcaaatatcacaaattttctttccttctctgcaagtgtcaataaatcagctagtgttggaattgactgatttcttgctctttctttatctgcctctgatagaggtttcatattgtaaaatggcctgagctctggttttacaaaccatttgcctgcattcagagtcgataggaaatcccagttgaagaaggcagggttctcgcaggcagattctggctgaacttccccaatattggttgttcttttcaggtcaaagtcatgcatgaggaaaggcacatgatcataacttaagtgtatatcagtctccaatccatgggctccatgttcaacagctttctcaaaggacatcatggtattctcaggccccaacatgggtgcacctctatgtccaaagatggttggcttgggccccaaattctccttctcctgaatgcagggagaataaatccccagtggcatcaaatagagacctcttaaccttgtgattacattacattgcttgagtctttttttctcagaatgtgtcatcctgtatcttctcattctaacttctctttccaaacatgccacgtagaaggccacaggccagaaaaggataaccatcacagttatgctgaccaggtgcacgtagggagcaaagatctgcattgacagcccagctaccagccacctttctttccagaatttgcatataatgaacattaaaatgacacacagaagaatcactagcagaatcaggatcttatgacacaagtgcaggtatagttcaatcctttcccaaagcaacaaaaatccaagtaacagtcaaagttaaagtattcactggatgtttctatccacaggaacagcaacatcagagacaagacaaatgaaattaccaggcacggcaaaataattgctctttctgggaaaagaaaaaagaaatctaacttagctccatttatccttgttacctcagcagtttctgtatacacttgccaaaggtcagcatagttgcactgccatgcattaccctcctgaggctggagtgatcactctcttctttttacccctaccaaatcctgtatatgcctatttacaacctttcttacacttaactggaattatgcatttatgttttatctgatgctacactgtttcttctttgaggaaaaggaacgtctctgtattaccaatacatagcattgtttcttgaatgcagctggctctcaacaatcatctgttgaattcatctgcctctccagctatcaaatgttttgttcagcaattaatttattgattcattcatcattaattggttcatttagtcatcaatctaccccattggagaagaaagggggaatcagagttaaagaataattttttttaagtagctattttgttctagtaaaatgctagggaatttcacaagctactttcatttgatttatttctcattagagccatatgagttgggcatcaacctcatttttgcagaagaaagctcagagaggtaaaataattgattcaagatcacacagctaagaagtggcaggggcaggactagaacccagatctgtgtaagctcaaagccaaaatggaggttatcattatggagaaggtactgctttctctgaaggcaaagaagtctccctgtgttagttttgtccttttcaatacgtcctccacacaatcaaataatcattccaaaacacagctcagactacttcatcagcttaaagtctttggggattctttattcccaacatggcagaagtcaaattcttaaaaccacacaacattggacccatctccctctctagcttcttttcccctcacttcttcacattcatatcctctccttcatctaaaataaaccttgtatcagtctccaaactcattatgccctttgactactcctccaataccaattcttccaccatccccaattctctacctatccaattcttaatcacccatcaccttctaaaaggtggccctccccttggtatgtgcctgtgtacatgcgcatacagttacagcacttctctcactatattgagattgtgtgtgtacttatctttccccacagtagactgaattccttgagagcaggaaccatgcctgaagcacttgtattatccccagtgactagcatagaggccgaatatctgggcaggaaagatacagtggggacagaagaacattccttcctactgcagggaaacctcccatttcctacccctttccttgtgttccccacctcaggtataagaaattaatgacccaactggtctgattctgggaccctagttggaccatgtttacaaataagtaaaggtacatgattttgctcttctgttctcatttcagtgtgctgatcatttaatcacttataccatgtagctcaccaaagggttccaacatatggcttacaaatagaggccctaaaaaaggctagtccacgtgccaccactcagccttactagagttcttcctcagggaaaatcaccactagcttgaccaataataaaggagcaccttgtttctcacttgctgtttttttctcttttatggaagaaatggagccctagcatccccagtcctggagaccataaagagccctcatggggcccagcagtcagcctatgctccccgcatctgagaaaatgtggtccagctccttatcagtctgtacccaagtgcagcaacaaaatccaactttagttttttcccattgtctgaatttccagaggcaactatagcagccagtaaggaaggtgacaaagcatttgtggttgaagatgcgtggaatccatggattaagcttttttggtttttctgtcttattcctcttgtgctcaatcctgttgaccttcttaaacatgattcaccctttagcgagacttcccagtcccaacccaaatccaatcttcacgcctgaggagaccagcgtctcttaagatggacgcctggctggaagggcagcccgaggg

SEQ ID NO: 18600 - RNA, 2051 nt, Homo sapiens
  source 1..2051: mol_type = other RNA
tgaggtagtagtttcttggatggtgctgcaaaattgaaatggccttggtgttcctttccactcttgggtagagccgggtagagggctgctagagtccaaggaccttccacaactcggacaggaggtttcatggctatgtgcaaatctatctatctatctatcttcctcattcttacttccactctgagtatctgtgcgagtgctggaggtttcaaacaatttttctttttcagtctctctccgccagtgaaaacaaaatatggcaacaataaaaagcacagaaatgatatctgcaaggagccacatgaacacatagaactttggtgtcatgaagaagtgagggtgatcaagctgactcaggagcccaatgttgtctgtggtcactgagttaatcctggagcaccaggccagtgagaaaagccaaggctcattgacggtgtatacgttgatatggatgttagctgctttataatctcttaacccattagggaacaacttcttgtagtcaacatttattatactgatattgtttttagcaagggtttcaatggatactaaacggcccacatgctgaaaaccaggagccacggacctgacgtattgcctatcatgagctggcaaccaaaaaatcagatgttgctcgattttagaggcaaggatcacgcttactacttggcggacaaatgtgtgtctgagaggatgttttggtggagggcgatgaagatcaaatatcacaaattttctttccttctctgcaagtgtcaataaatcagctagtgttggaattgactgatttcttgctctttctttatctgcctctgatagaggtttcatattgtaaaatggcctgagctctggttttacaaaccatttgcctgcattcagagtcgataggaaatcccagttgaagaaggcagggttctcgcaggcagattctggctgaacttccccaatattggttgttcttttcaggtcaaagtcatgcatgaggaaaggcacatgatcataacttaagtgtatatcagtctccaatccatgggctccatgttcaacagctttctcaaaggacatcatggtattctcaggccccaacatgggtgcacctctatgtccaaagatggttggcttgggccccaaattctccttctcctgaatgcagggagaataaatccccagtggcatcaaatagagacctaaaaggataagaagaaagggtaatccaacaggcacttgtagacctcttaaccttgtgattacattacattgcttgagtctttttttctcagaatgtgtcatcctgtatcttctcattctaacttctctttccaaacatgccacgtagaaggccacaggccagaaaaggataaccatcacagttatgctgaccaggtgcacgtagggagcaaagatctgcattgacagcccagctaccagccacctttctttccagaatttgcatataatgaacattaaaatgacacacagaagaatcactagcagaatcaggatcttatgacacaagtgcaggtatagttcaatcctttcccaaagcaacaaaaatccaagtaacaacagcaatgaagagtaggcagtcaggatcctagctaaactcagaataaaaatagaccagaaaaaccagtatcctgttcctagaaaagtgacccagtcaaagttaaagtattcactggatgtttctatccacaggaacagcaacatcagagacaagacaaatgaaattaccaggcacggcaaaataattgctctttccaagtgcagcaacaaaatccaactttagttttttcccattgtctgaatttccagaggcaactatagcagccagtaaggaaggtgacaaagcatttgtggttgaagatgcgtggaatccatggattaagcttttttggtttttctgtcttattcctcttgtgctcaatcctgttgaccttcttaaacatgattcaccctttagcgagacttcccagtcccaacccaaatccaatcttcacgcctgaggagaccagcgtctcttaagatggacgcctggctggaag

SEQ ID NO: 18601 - RNA, 2162 nt, Homo sapiens
  source 1..2162: mol_type = other RNA
tgaggtagtagtttcttggatggtgctgcaaaattgaaatggccttggtgttcctttccactcttgggtagagccgggtagagggctgctagagtccaaggaccttccacaactcggacaggaggtttcatggctatgtgcaaatttccactctgagtatctgtgcgagtgctggaggtttcaaacaatttttctttttcagtctctctccgccagtgaaaacaaaatatggcaacaataaaaagcacagaaatgatatctgcaaggagccacatgaacacatagaactttggtgtcatgaagaagtgagggtgatcaagctgactcaggagcccaatgttgtctgtggtcactgagttaatcctggagcaccaggccagtgagaaaagccaaggctcattgacggtgtatacgttgatatggatgttagctgctttataatctcttaacccattagggaacaacttcttgtagtcaacatttattatactgatattgtttttagcaagggtttcaatggatactaaacggcccacatgctgaaaaccaggagccacggacctgacgtattgcctatcatgagctggcaaccaaaaaatcagatgttgctcgattttagaggcaaggatcacgcttactacttggcggacaaatgtgtgtctgagaggatgttttggtggagggcgatgaagatcaaatatcacaaattttctttccttctctgcaagtgtcaataaatcagctagtgttggaattgactgatttcttgctctttctttatctgcctctgatagaggtttcatattgtaaaatggcctgagctctggttttacaaaccatttgcctgcattcagagtcgataggaaatcccagttgaagaaggcagggttctcgcaggcagattctggctgaacttccccaatattggttgttcttttcaggtcaaagtcatgcatgaggaaaggcacatgatcataacttaagtgtatatcagtctccaatccatgggctccatgttcaacagctttctcaaaggacatcatggtattctcaggccccaacatgggtgcacctctatgtccaaagatggttggcttgggccccaaattctccttctcctgaatgcagggagaataaatccccagtggcatcaaatagagacctaaaaggataagaagaaagggtaatccaacaggcacttgtagacctcttaaccttgtgattacattacattgcttgagtctttttttctcagaatgtgtcatcctgtatcttctcattctaacttctctttccaaacatgccacgtagaaggccacaggccagaaaaggataaccatcacagttatgctgaccaggtgcacgtagggagcaaagatctgcattgacagcccagctaccagccacctttctttccagaatttgcatataatgaacattaaaatgacacacagaagaatcactagcagaatcaggatcttatgacacaagtgcaggtatagttcaatcctttcccaaagcaacaaaaatccaagtaacaacagcaatgaagagtaggcagtcaggatcctagctaaactcagaataaaaatagaccagaaaaaccagtatcctgttcctagaaaagtgacccagtcaaagttaaagtattcactggatgtttctatccacaggaacagcaacatcagagacaagacaaatgaaattaccaggcacggcaaaataattgctctttttttatggaagaaatggagccctagcatccccagtcctggagaccataaagagccctcatggggcccagcagtcagcctatgctccccgcatctgagaaaatgtggtccagctccttatcagtctgtacccaagtgcagcaacaaaatccaactttagttttttcccattgtctgaatttccagaggcaactatagcagccagtaaggaaggtgacaaagcatttgtggttgaagatgcgtggaatccatggattaagcttttttggtttttctgtcttattcctcttgtgctcaatcctgttgaccttcttaaacatgattcaccctttagcgagacttcccagtcccaacccaaatccaatcttcacgcctgaggagaccagcgtctcttaagatggacgcctggctggaagggcagcccgaggg

SEQ ID NO: 18602 - RNA, 1109 nt, Homo sapiens
  source 1..1109: mol_type = other RNA
tgaggtagtagtttctttcagaaggaaaatgagctgtgcaggtcatatgagggtcttcttatcctattatgatatctctagtaactctggcagtaacagaagcaaagtaaatctggacatgacagacatttagacgaatctggcagtacactgagttttaactggacaccaagcaggcaaggctggaaggttttgctctctttgtgctaaaggttttgaaaaccttgaaggagaatcattttgacaagaagtactgtgtagtctgctgcagtcttctcttgggtccaactggcactgcctgttagtctattgggaggcccagcaggtcacaactgacgtcccacagccgccttgctatagtctcattacgagcttgggcagagacccatgccacatgacagtcactgaaatgattcccacttagaatctcaagaccttctgttaaggcacagtgcaggctggtctgggctccctgctgaggagtcttgatgaaaaaggagaaaagccaccacatccatctcatgaaagatgagtgccgaaccagttcagattggactgtgccagggtgtacagaatacgtcgtaacgccagagcccaagtggttgactcctatgtgcatctcaaagccatctgctgtcttcgagtacggacacatcatcactcctgcattgttgatcaaaacgtggaggtgcttttcctcagctaagaagcccttagcaaaagctcgaatagacttagtatcagacaggtccagtttccgcaccaacacctgctggttccctgtcgtggtctggatctctttggccaccaattcccccttttccacatcccggcaagctaaatatactcgagctcctctctgagccagctctttggctgtctccttcccgatacctgtattagctcctgtgaccacaactactttcccaggaagctgaacagttgatgtacacaccccactggacagcattttcctgatttggggcgcagccatatacagaaggaagggcagaaggaggagcaacagcgggaacatgagctcaaccatctctgccggctgcagcggcaccagagcgggatgctccagcgttgctcgccgactatggctt

SEQ ID NO: 18603 - RNA, 1319 nt, Homo sapiens
  source 1..1319: mol_type = other RNA
tgaggtagtagtttctttcagaaggaaaatgagctgtgcaggtcatatgagggtcttcttatcctattatgatatctctagtaactctggcagtaacagaagcaaagtaaatctggacatgacagacatttagacgaatctggcagtacactgagttttaactggacaccaagcaggcaaggctggaaggttttgctctctttgtgctaaaggttttgaaaaccttgaaggagaatcattttgacaagaagtactgtgtagtctgctgcagtcttctcttgggtccaactggcactgcctgttagtctattgggaggcccagcaggtcacaactgacgtcccacagccgccttgctatagtctcattacgagcttgggcagagacccatgccacatgacagtcactgaaatgattcccacttagaatctcaagaccttctgttaaggcacagtgcaggctggtctgggctccctgctgaggagtcttgatgaaaaaggagaaaagccaccacatccatctcatgaaagatgagtgccgaaccagttcagattggactgtgccagggtgtacagaatacgtcgtaacgccagagccttttagtctccgggccagttcctgggtgaagaggatgttggctagcttgctgtgacagtaggccaggcctgcattgtagaatttctcgccctgcaggttatggaagtggatccttcccaggtgatgtgcgagggaagacacatttactatccttgatggggctgattcctttagtttctctagcagcagatgggttaggaggaagtgacccaagtggttgactcctatgtgcatctcaaagccatctgctgtcttcgagtacggacacatcatcactcctgcattgttgatcaaaacgtggaggtgcttttcctcagctaagaagcccttagcaaaagctcgaatagacttagtatcagacaggtccagtttccgcaccaacacctgctggttccctgtcgtggtctggatctctttggccaccaattcccccttttccacatcccggcaagctaaatatactcgagctcctctctgagccagctctttggctgtctccttcccgatacctgtattagctcctgtgaccacaactactttcccaggaagctgaacagttgatgtacacaccccactggacagcattttcctgatttggggcgcagccatatacagaaggaagggcagaaggaggagcaacagcgggaacatgagctcaaccatctctgccggctgcagcggcaccagagcgggatgctccagcgttgctcgccgactatggctt

SEQ ID NO: 18604 - RNA, 279 nt, Homo sapiens
  source 1..279: mol_type = other RNA
tgaggtagtagtttgtacagttaactggttcttgcgtagcgtcatttatttttggatctcgcctccatgggggggtgttctccacagaggatattgtcccactttgaggtcctcgcacttaagcgactcctcgcccccggcggaggtggcaacagccccccagggtcctgtagtgactgagacgaaccacaggacaccaacgagtctggccgtcacggcctccggagcagacggaccagacggccaggcggccgccatcttggagaccgacactttctc

SEQ ID NO: 18605 - RNA, 256 nt, Homo sapiens
  source 1..256: mol_type = other RNA
tgaggtagtagtttgtacagttaactggttcttgcgtagcgtcatttatttttggatctttacaaatatattgtcccactttgaggtcctcgcacttaagcgactcctcgcccccggcggaggtggcaacagccccccagggtcctgtagtgactgagacgaaccacaggacaccaacgagtctggccgtcacggcctccggagcagacggaccagacggccaggcggccgccatcttggagaccgacactttctc

SEQ ID NO: 18606 - RNA, 1542 nt, Homo sapiens
  source 1..1542: mol_type = other RNA
tgagtaccgccatgtctgttggggatgctggggggctggggtaggggtttggggttgggtctggggctgtgggggcagctggggctgtggttgtgattgtggctggggctgtggttgtggttggggctgcagcttaggcgggggtgctcgggtgaagaggggggacccagggagcatggcgcggctggccccgtgctcccagaaggcgttctgcagcttgaagatcatgctgagggggatgggacgctggcgcggggccccgcggggctgggggctggaggggggcatggggatgcggctgacgggctgccagctgcgaggcaaagtgcccgacggccccgcggagcccagcgagcgccggtagctgcccgcgtctgaacgccggtcgctggccagaggagagaccttgtaattgcgcggcagggtggcgctagtgaggttgtccttgccggtgccccccagtccatccaggctgctctccctccaaggcaacagctgcaggctcggcgaggcaggccttgcgaagacgtccaggcgttcatagctcgctgtctgcgaaggcttcttctcgtacgccacgtccaggtcagactcgttccaggctttcggaggccgccggcgcagcgtcaggtcgtcttgcgcgcgcagaggcggggcgaatgcgctgccgccggagcctagcagggagctcccgaaggcggacgctggcgcgtcgtaggctgtggcaggggggcgcggtgacggcccacgctcggggaagaaggcctggggcccctccgccagggggctgccgcggggggagcctgcgcggcccaggaagtcgaaaggcgtggggggaccctgctggcggagcgggcctggcccgggccgcggggagggcgcacggccgagggagctgcctgcgccatcgaaggcgcggggccggggcgaggtcgcgcggtccaggctgccgtaggcgtccggctgcaggtagagcggggtgcgcggcgacgacggccgtcccttgggggacagcgggctgtaggggtgtagggttggggcactctctgatcgtccgaacggggtgtctgcgccgtcggtggccgccttccggggggaccctcggctgccgaagggctcagggatcgagctggagctgtaccggggcggcctagaagggggtccggcctgcgggccaggaggcgcgggagagtctgaccacagcgactccagctgcttggtcagttcatccaccttggccgccgccgtgtccagctccatctgcttcagatccatgtgtttcatggccagcgactggaagttcatgtccagaaagtcccgcgcgctctggaatgcctcgctgtccatggtgccggccggagcgggcgcctcagtctcgtaatccgtaaaatggggatgaaagttcacctcataggactactgtaagaatccacctggtcagaaggtgcaggaagaattcagagctctgagaattgaggcctcaggaagaagagactgtctcttcaagaatttcagaccaatcgaccgtcctgtctctttaag

SEQ ID NO: 18607 - RNA, 1426 nt, Homo sapiens
  source 1..1426: mol_type = other RNA
tgagtaccgccatgtctgttggggatgctggggggctggggtaggggtttggggttgggtctggggctgtgggggcagctggggctgtggttgtgattgtggctggggctgtggttgtggttggggctgcagcttaggcgggggtgctcgggtgaagaggggggacccagggagcatggcgcggctggccccgtgctcccagaaggcgttctgcagcttgaagatcatgctgagggggatgggacgctggcgcggggccccgcggggctgggggctggaggggggcatggggatgcggctgacgggctgccagctgcgaggcaaagtgcccgacggccccgcggagcccagcgagcgccggtagctgcccgcgtctgaacgccggtcgctggccagaggagagaccttgtaattgcgcggcagggtggcgctagtgaggttgtccttgccggtgccccccagtccatccaggctgctctccctccaaggcaacagctgcaggctcggcgaggcaggccttgcgaagacgtccaggcgttcatagctcgctgtctgcgaaggcttcttctcgtacgccacgtccaggtcagactcgttccaggctttcggaggccgccggcgcagcgtcaggtcgtcttgcgcgcgcagaggcggggcgaatgcgctgccgccggagcctagcagggagctcccgaaggcggacgctggcgcgtcgtaggctgtggcaggggggcgcggtgacggcccacgctcggggaagaaggcctggggcccctccgccagggggctgccgcggggggagcctgcgcggcccaggaagtcgaaaggcgtggggggaccctgctggcggagcgggcctggcccgggccgcggggagggcgcacggccgagggagctgcctgcgccatcgaaggcgcggggccggggcgaggtcgcgcggtccaggctgccgtaggcgtccggctgcaggtagagcggggtgcgcggcgacgacggccgtcccttgggggacagcgggctgtaggggtgtagggttggggcactctctgatcgtccgaacggggtgtctgcgccgtcggtggccgccttccggggggaccctcggctgccgaagggctcagggatcgagctggagctgtaccggggcggcctagaagggggtccggcctgcgggccaggaggcgcgggagagtctgaccacagcgactccagctgcttggtcagttcatccaccttggccgccgccgtgtccagctccatctgcttcagatccatgtgtttcatggccagcgactggaagttcatgtccagaaagtcccgcgcgctctggaatgcctcgctgtccatggtgccggccggagcgggcgcctgtctcttcaagaatttcagaccaatcgaccgtcctgtctctttaaggcttaggaag

SEQ ID NO: 18608 - RNA, 1438 nt, Homo sapiens
  source 1..1438: mol_type = other RNA
tgagtaccgccatgtctgttggggatgctggggggctggggtaggggtttggggttgggtctggggctgtgggggcagctggggctgtggttgtgattgtggctggggctgtggttgtggttggggctgcagcttaggcgggggtgctcgggtgaagaggggggacccagggagcatggcgcggctggccccgtgctcccagaaggcgttctgcagcttgaagatcatgctgagggggatgggacgctggcgcggggccccgcggggctgggggctggaggggggcatggggatgcggctgacgggctgccagctgcgaggcaaagtgcccgacggccccgcggagcccagcgagcgccggtagctgcccgcgtctgaacgccggtcgctggccagaggagagaccttgtaattgcgcggcagggtggcgctagtgaggttgtccttgccggtgccccccagtccatccaggctgctctccctccaaggcaacagctgcaggctcggcgaggcaggccttgcgaagacgtccaggcgttcatagctcgctgtctgcgaaggcttcttctcgtacgccacgtccaggtcagactcgttccaggctttcggaggccgccggcgcagcgtcaggtcgtcttgcgcgcgcagaggcggggcgaatgcgctgccgccggagcctagcagggagctcccgaaggcggacgctggcgcgtcgtaggctgtggcaggggggcgcggtgacggcccacgctcggggaagaaggcctggggcccctccgccagggggctgccgcggggggagcctgcgcggcccaggaagtcgaaaggcgtggggggaccctgctggcggagcgggcctggcccgggccgcggggagggcgcacggccgagggagctgcctgcgccatcgaaggcgcggggccggggcgaggtcgcgcggtccaggctgccgtaggcgtccggctgcaggtagagcggggtgcgcggcgacgacggccgtcccttgggggacagcgggctgtaggggtgtagggttggggcactctctgatcgtccgaacggggtgtctgcgccgtcggtggccgccttccggggggaccctcggctgccgaagggctcagggatcgagctggagctgtaccggggcggcctagaagggggtccggcctgcgggccaggaggcgcgggagagtctgaccacagcgactccagctgcttggtcagttcatccaccttggccgccgccgtgtccagctccatctgcttcagatccatgtgtttcatggccagcgactggaagttcatgtccagaaagtcccgcgcgctctggaatgcctcgctgtccatggtgccggccggagcgggcgcctgtctcttcaagaatttcagaccaatcgaccgtcctgtctctttaaggcttaggaagagcagtgtggct

SEQ ID NO: 18609 - RNA, 1439 nt, Homo sapiens
  source 1..1439: mol_type = other RNA
tgagtaccgccatgtctgttggggatgctggggggctggggtaggggtttggggttgggtctggggctgtgggggcagctggggctgtggttgtgattgtggctggggctgtggttgtggttggggctgcagcttaggcgggggtgctcgggtgaagaggggggacccagggagcatggcgcggctggccccgtgctcccagaaggcgttctgcagcttgaagatcatgctgagggggatgggacgctggcgcggggccccgcggggctgggggctggaggggggcatggggatgcggctgacgggctgccagctgcgaggcaaagtgcccgacggccccgcggagcccagcgagcgccggtagctgcccgcgtctgaacgccggtcgctggccagaggagagaccttgtaattgcgcggcagggtggcgctagtgaggttgtccttgccggtgccccccagtccatccaggctgctctccctccaaggcaacagctgcaggctcggcgaggcaggccttgcgaagacgtccaggcgttcatagctcgctgtctgcgaaggcttcttctcgtacgccacgtccaggtcagactcgttccaggctttcggaggccgccggcgcagcgtcaggtcgtcttgcgcgcgcagaggcggggcgaatgcgctgccgccggagcctagcagggagctcccgaaggcggacgctggcgcgtcgtaggctgtggcaggggggcgcggtgacggcccacgctcggggaagaaggcctggggcccctccgccagggggctgccgcggggggagcctgcgcggcccaggaagtcgaaaggcgtggggggaccctgctggcggagcgggcctggcccgggccgcggggagggcgcacggccgagggagctgcctgcgccatcgaaggcgcggggccggggcgaggtcgcgcggtccaggctgccgtaggcgtccggctgcaggtagagcggggtgcgcggcgacgacggccgtcccttgggggacagcgggctgtaggggtgtagggttggggcactctctgatcgtccgaacggggtgtctgcgccgtcggtggccgccttccggggggaccctcggctgccgaagggctcagggatcgagctggagctgtaccggggcggcctagaagggggtccggcctgcgggccaggaggcgcgggagagtctgaccacagcgactccagctgcttggtcagttcatccaccttggccgccgccgtgtccagctccatctgcttcagatccatgtgtttcatggccagcgactggaagttcatgtccagaaagtcccgcgcgctctggaatgcctcgctgtccatggtgccggccggagcgggcgcggatccgggcagatcctggcacctgggggcttcctccagctcgggctccggcttggggagcggagaacggg

SEQ ID NO: 18610 - RNA, 1482 nt, Homo sapiens
  source 1..1482: mol_type = other RNA
tgagtaccgccatgtctgttggggatgctggggggctggggtaggggtttggggttgggtctggggctgtgggggcagctggggctgtggttgtgattgtggctggggctgtggttgtggttggggctgcagcttaggcgggggtgctcgggtgaagaggggggacccagggagcatggcgcggctggccccgtgctcccagaaggcgttctgcagcttgaagatcatgctgagggggatgggacgctggcgcggggccccgcggggctgggggctggaggggggcatggggatgcggctgacgggctgccagctgcgaggcaaagtgcccgacggccccgcggagcccagcgagcgccggtagctgcccgcgtctgaacgccggtcgctggccagaggagagaccttgtaattgcgcggcagggtggcgctagtgaggttgtccttgccggtgccccccagtccatccaggctgctctccctccaaggcaacagctgcaggctcggcgaggcaggccttgcgaagacgtccaggcgttcatagctcgctgtctgcgaaggcttcttctcgtacgccacgtccaggtcagactcgttccaggctttcggaggccgccggcgcagcgtcaggtcgtcttgcgcgcgcagaggcggggcgaatgcgctgccgccggagcctagcagggagctcccgaaggcggacgctggcgcgtcgtaggctgtggcaggggggcgcggtgacggcccacgctcggggaagaaggcctggggcccctccgccagggggctgccgcggggggagcctgcgcggcccaggaagtcgaaaggcgtggggggaccctgctggcggagcgggcctggcccgggccgcggggagggcgcacggccgagggagctgcctgcgccatcgaaggcgcggggccggggcgaggtcgcgcggtccaggctgccgtaggcgtccggctgcaggtagagcggggtgcgcggcgacgacggccgtcccttgggggacagcgggctgtaggggtgtagggttggggcactctctgatcgtccgaacggggtgtctgcgccgtcggtggccgccttccggggggaccctcggctgccgaagggctcagggatcgagctggagctgtaccggggcggcctagaagggggtccggcctgcgggccaggaggcgcgggagagtctgaccacagcgactccagctgcttggtcagttcatccaccttggccgccgccgtgtccagctccatctgcttcagatccatgtgtttcatggccagcgactggaagttcatgtccagaaagtcccgcgcgctctggaatgcctcgctgtccatggtgccggccggagcgggcgcggatccgggcagatcctggcacctgggggcttcctccagctcgggctccggcttggggagcggagaacggggcggggcaggagctgtctcttcaagaatttcagaccaatcgac

SEQ ID NO: 18611 - RNA, 4206 nt, Homo sapiens
  source 1..4206: mol_type = other RNA
tgagtgacaggggaaatggggagaagagagagaagaggagaggagacagaagcagagacagggagagggagagaaacagaaaacatgttagacagagggggtggggggagctgtatacagacagacagacatggagaggtgggatcgtgttgagagagatcaggaaggtctcgatgggcaagagatgcagagaagacaagaggttccaagagcacgtgcacggagttgggtgcgatacccacgagaaagaacatcggagttactggacagggaactgaggatcttggaagctctgaccaggcaaagagggagagactgtgacctagagacagaagcacgtgagcaaatatgagaacgtgcacgagaacaagcgagaagaaccagtcacacaaaacacccatgaagaaagcaacacgactaaggacagacacaggaagtcccaggtccagcagctcagggaggaaggcagggaaggaggagaagcaccgagctgagaaatgggtaagaaggggctgccccattttgggccgcagaggagaaaggggcaaaggaggtggccagaaagggcctgacaagttcaaccggccagcagctaccaccctgaccagatccgcattccagcccggcccctcacacactcagctcccactccaggcccacactcaatcctgctgccacagccttcatactccgcctggttgcccccagctcagcaccccctactgtggagggtctgcagccccgtcccccaacccactagggtaatgcctgatgcaggagagcaatttggtcccctgcagccatggttgggagaaaaggcaagggatgaggagaccaagggcctggaaactaagacctctggaaggaacccgcaaacaggcgctctgtgggaccaagaagttcggtgaagttctacaggggcccagaccccagagccggtggtggtcatggtgcaatgaagctatgaaggcagagagcatgaggctggaggagtgagggggctgagataacggagatggggtgaagaggtcatggagccgggccgagggtcagcctgggggcataccggggaggctaggcggcaggacaaagcagacagaggcagcctgggccaaaggcacagttccgctcagatattttatttgtgtttgtcttttttttgaggctcttgggctgctggcgaacctgggccgcatgcttctgccgcaactcttgctcacgccgcttgttgtactccagctggttgcccagctccgtctggtgctgcaggcgggtgagctcagcccgcgtgcgctgcacggcctggagctgccgcagctccagctcccgcgtggcctcgtgctgccgaagcagcagtgcacactccaagtccttctgggtctgcttcttgttcaggtcctcccgcagcaggtcctggtccaggctgtgccgagccagcaacatcttgcgcttgtactggcgacactgcagctcaaagtactggcgctgccgccgcagcagccctgcttcctcctccgcctggcactgctggagctgctccttctgccgcagcagccactcggccttctcccgcttgggagtgctggggttctcctggagctcctccttcagctgttccttgcgaagtttgtaggtccgcttctgtgcctccagcagggcagccagctccttcttctgctgcccaaggatgtgctgctggaacttccgctcctcggcctgggcagctcgtgcctccttctcacctatggcctggtgccgccgggccagcttttctgcctctgccccaaagccagcccgctgcgcctcaagctcccgctgcagccgtgcactgtgctcctcccgttcacccctcagccgtgactccagggccagcagctgcttctggtgctgtcgtcgcatccgcttatagccgctcagctgctcccgcagcgcagagtcctgctcatgctcctggatctgacggctgaccagggaggcggttcggatggtggcaaagtggtctcggttacggcagtaggcccggcggcgggcggaagaggtggtggaagtgggagctggggctgcaggcggctggagagggctgggggttatctctggctggtaggggtcatcatataggttgtcagagcccggcagccggtggataatggagctgtgagaggtgactgtgtgctccccctcctgcatcatggccatctcccgggcttcagggccttcttcctcctcctcctcttcctcctcctcctcctcctcttcctcgttgtctgaggcatctgctaggctgttgacggagctgctctggctggaggcgctgatggacatgctgggcactgagtggctactctcgaggctggtcagagtcccggcccggtgcatgtagggctcggcctcctcttcctcctctggggcctcggcaccagggccgttgggtgcctcttggaacaggatcttcttcatcttgcggtactgcaggttgtccagctcccgcacggcatccttggtcctctggatcaggtccatgatgactgtgggtggccgctcccggagcacaaagcggtgcttcaggagaacctctgaggttggtctgtcttgagggattttctgaagacaggagtcgacaaaattccggaagtactcagaccagtgtcctgactggagcacgggggattcgttctgtgcaatgtggtataaggcactcatcgcattcatgttaaagagcggtggtttccgttcagccagctcgatgcaggttatccccaaggaccagacgtccactttgccatcgtactgcccctcatccatggccaggatcacctcgggtgccatccagtatggggtgcccacgaaggagttggcaggtgccatgatggacgcagaaccaaagtcccctagcttcactaaccctggctctgacagcaggatgtttccagccttcacatccctatggatcatgttgtgggagtgcagatatgccaggccctgaagcgccccgtgggtcacagctgcgatctctacctcctgaaggggtttcttgtgcacttctagaaggtcagaagctgagcccaggcaatactccattaccagccaagccgtgtgctccctcaggtaacagccccggtactgaatggtgttgggatgccggagcttctgtaagaaccgcacctccttgatgatgtcttgccatttctcattggactgcttcccactgtaggacatcttcttgatggccaccacctcactattccggacatcccgggcaaagtatacggctccaaagctgccatggccaatttcccggaggtcagagaagagcttttctgggtcatccttgaagaagagctcagccacatctgggtccttcaggctcccggcccggcccccagctggcatggtggcccctgggggccctgagagtggggcctggcctggtaggggtcactatggtgccccagcgcctccgcttccgcctggggtcctccagcggctctgccaagcagggagaggggcaaggagacctttccccttgccacctcttcctcggctttcgcccttcctgaggggcgggcccgggaagcctcccctggaggggagggggtgacaacctaatctgacctcgcggtccagtcctccccctcgtcgagggcgacagctgccgaattccggatttctgattgtggggtctgaaccccgaatatctgaacgggatggagactgaatccgatatttgaacgcccggggaatgaaccccggatactggtgcacgcaggggcctgaacctgatatttgaaattctatgaaacagagacccaggtttagagaggttgggacccgagtcccggatatctggactatgaggactgttacccgggtatctgagaaaggaggaggggcaaagcctggaaatttgggacccaggggcctgagctgtaggtcttcggccaccgactgggggcccaccccgaggacgtccggccgcacggcccctctcacgccggggtccgagggtgacagcccccactcccgccccggcctcctccctctcccttctctcttccgagaatagctgaacgattgtagctaaggtgctgctgacggtccccgcgccctctctgcctctcctcttctccgtctcagcctctctccgcaccacagccccggtctcgtcccggtctccctctccctcttcctcccaattccaagatggag

SEQ ID NO: 18612 - RNA, 4227 nt, Homo sapiens
  source 1..4227: mol_type = other RNA
tgagtgacaggggaaatggggagaagagagagaagaggagaggagacagaagcagagacagggagagggagagaaacagaaaacatgttagacagagggggtggggggagctgtatacagacagacagacatggagaggtgggatcgtgttgagagagatcaggaaggtctcgatgggcaagagatgcagagaagacaagaggttccaagagcacgtgcacggagttgggtgcgatacccacgagaaagaacatcggagttactggacagggaactgaggatcttggaagctctgaccaggcaaagagggagagactgtgacctagagacagaagcacgtgagcaaatatgagaacgtgcacgagaacaagcgagaagaaccagtcacacaaaacacccatgaagaaagcaacacgactaaggacagacacaggaagtcccaggtccagcagctcagggaggaaggcagggaaggaggagaagcaccgagctgagaaatgggtaagaaggggctgccccattttgggccgcagaggagaaaggggcaaaggaggtggccagaaagggcctgacaagttcaaccggccagcagctaccaccctgaccagatccgcattccagcccggcccctcacacactcagctcccactccaggcccacactcaatcctgctgccacagccttcatactccgcctggttgcccccagctcagcaccccctactgtggagggtctgcagccccgtcccccaacccactagggtaatgcctgatgcaggagagcaatttggtcccctgcagccatggttgggagaaaaggcaagggatgaggagaccaagggcctggaaactaagacctctggaaggaacccgcaaacaggcgctctgtgggaccaagaagttcggtgaagttctacaggggcccagaccccagagccggtggtggtcatggtgcaatgaagctatgaaggcagagagcatgaggctggaggagtgagggggctgagataacggagatggggtgaagaggtcatggagccgggccgagggtcagcctgggggcataccggggaggctaggcggcaggacaaagcagacagaggcagcctgggccaaaggcacagttccgctcagatattttatttgtgtttgtcttttttttgaggctcttgggctgctggcgaacctgggccgcatgcttctgccgcaactcttgctcacgccgcttgttgtactccagctggttgcccagctccgtctggtgctgcaggcgggtgagctcagcccgcgtgcgctgcacggcctggagctgccgcagctccagctcccgcgtggcctcgtgctgccgaagcagcagtgcacactccaagtccttctgggtctgcttcttgttcaggtcctcccgcagcaggtcctggtccaggctgtgccgagccagcaacatcttgcgcttgtactggcgacactgcagctcaaagtactggcgctgccgccgcagcagccctgcttcctcctccgcctggcactgctggagctgctccttctgccgcagcagccactcggccttctcccgcttgggagtgctggggttctcctggagctcctccttcagctgttccttgcgaagtttgtaggtccgcttctgtgcctccagcagggcagccagctccttcttctgctgcccaaggatgtgctgctggaacttccgctcctcggcctgggcagctcgtgcctccttctcacctatggcctggtgccgccgggccagcttttctgcctctgccccaaagccagcccgctgcgcctcaagctcccgctgcagccgtgcactgtgctcctcccgttcacccctcagccgtgactccagggccagcagctgcttctggtgctgtcgtcgcatccgcttatagccgctcagctgctcccgcagcgcagagtcctgctcatgctcctggatctgacggctgaccagggaggcggttcggatggtggcaaagtggtctcggttacggcagtaggcccggcggcgggcggaagaggtggtggaagtgggagctggggctgcaggcggctggagagggctgggggttatctctggctggtaggggtcatcatataggttgtcagagcccggcagccggtggataatggagctgtgagaggtgactgtgtgctccccctcctgcatcatggccatctcccgggcttcagggccttcttcctcctcctcctcttcctcctcctcctcctcctcttcctcgttgtctgaggcatctgctaggctgttgacggagctgctctggctggaggcgctgatggacatgctgggcactgagtggctactctcgaggctggtcagagtcccggcccggtgcatgtagggctcggcctcctgcgaacagggcgtaggctgctcttcctcctctggggcctcggcaccagggccgttgggtgcctcttggaacaggatcttcttcatcttgcggtactgcaggttgtccagctcccgcacggcatccttggtcctctggatcaggtccatgatgactgtgggtggccgctcccggagcacaaagcggtgcttcaggagaacctctgaggttggtctgtcttgagggattttctgaagacaggagtcgacaaaattccggaagtactcagaccagtgtcctgactggagcacgggggattcgttctgtgcaatgtggtataaggcactcatcgcattcatgttaaagagcggtggtttccgttcagccagctcgatgcaggttatccccaaggaccagacgtccactttgccatcgtactgcccctcatccatggccaggatcacctcgggtgccatccagtatggggtgcccacgaaggagttggcaggtgccatgatggacgcagaaccaaagtcccctagcttcactaaccctggctctgacagcaggatgtttccagccttcacatccctatggatcatgttgtgggagtgcagatatgccaggccctgaagcgccccgtgggtcacagctgcgatctctacctcctgaaggggtttcttgtgcacttctagaaggtcagaagctgagcccaggcaatactccattaccagccaagccgtgtgctccctcaggtaacagccccggtactgaatggtgttgggatgccggagcttctgtaagaaccgcacctccttgatgatgtcttgccatttctcattggactgcttcccactgtaggacatcttcttgatggccaccacctcactattccggacatcccgggcaaagtatacggctccaaagctgccatggccaatttcccggaggtcagagaagagcttttctgggtcatccttgaagaagagctcagccacatctgggtccttcaggctcccggcccggcccccagctggcatggtggcccctgggggccctgagagtggggcctggcctggtaggggtcactatggtgccccagcgcctccgcttccgcctggggtcctccagcggctctgccaagcagggagaggggcaaggagacctttccccttgccacctcttcctcggctttcgcccttcctgaggggcgggcccgggaagcctcccctggaggggagggggtgacaacctaatctgacctcgcggtccagtcctccccctcgtcgagggcgacagctgccgaattccggatttctgattgtggggtctgaaccccgaatatctgaacgggatggagactgaatccgatatttgaacgcccggggaatgaaccccggatactggtgcacgcaggggcctgaacctgatatttgaaattctatgaaacagagacccaggtttagagaggttgggacccgagtcccggatatctggactatgaggactgttacccgggtatctgagaaaggaggaggggcaaagcctggaaatttgggacccaggggcctgagctgtaggtcttcggccaccgactgggggcccaccccgaggacgtccggccgcacggcccctctcacgccggggtccgagggtgacagcccccactcccgccccggcctcctccctctcccttctctcttccgagaatagctgaacgattgtagctaaggtgctgctgacggtccccgcgccctctctgcctctcctcttctccgtctcagcctctctccgcaccacagccccggtctcgtcccggtctccctctccctcttcctcccaattccaagatggag

SEQ ID NO: 18613 - RNA, 3391 nt, Homo sapiens
  source 1..3391: mol_type = other RNA
tgagtgacaggggaaatggggagaagagagagaagaggagaggagacagaagcagagacagggagagggagagaaacagaaaacatgttagacagagggggtggggggagctgtatacagacagacagacatggagaggtgggatcgtgttgagagagatcaggaaggtctcgatgggcaagagatgcagagaagacaagaggttccaagagcacgtgcacggagttgggtgcgatacccacgagaaagaacatcggagttactggacagggaactgaggatcttggaagctctgaccaggcaaagagggagagactgtgactttgaggctcttgggctgctggcgaacctgggccgcatgcttctgccgcaactcttgctcacgccgcttgttgtactccagctggttgcccagctccgtctggtgctgcaggcgggtgagctcagcccgcgtgcgctgcacggcctggagctgccgcagctccagctcccgcgtggcctcgtgctgccgaagcagcagtgcacactccaagtccttctgggtctgcttcttgttcaggtcctcccgcagcaggtcctggtccaggctgtgccgagccagcaacatcttgcgcttgtactggcgacactgcagctcaaagtactggcgctgccgccgcagcagccctgcttcctcctccgcctggcactgctggagctgctccttctgccgcagcagccactcggccttctcccgcttgggagtgctggggttctcctggagctcctccttcagctgttccttgcgaagtttgtaggtccgcttctgtgcctccagcagggcagccagctccttcttctgctgcccaaggatgtgctgctggaacttccgctcctcggcctgggcagctcgtgcctccttctcacctatggcctggtgccgccgggccagcttttctgcctctgccccaaagccagcccgctgcgcctcaagctcccgctgcagccgtgcactgtgctcctcccgttcacccctcagccgtgactccagggccagcagctgcttctggtgctgtcgtcgcatccgcttatagccgctcagctgctcccgcagcgcagagtcctgctcatgctcctggatctgacggctgaccagggaggcggttcggatggtggcaaagtggtctcggttacggcagtaggcccggcggcgggcggaagaggtggtggaagtgggagctggggctgcaggcggctggagagggctgggggttatctctggctggtaggggtcatcatataggttgtcagagcccggcagccggtggataatggagctgtgagaggtgactgtgtgctccccctcctgcatcatggccatctcccgggcttcagggccttcttcctcctcctcctcttcctcctcctcctcctcctcttcctcgttgtctgaggcatctgctaggctgttgacggagctgctctggctggaggcgctgatggacatgctgggcactgagtggctactctcgaggctggtcagagtcccggcccggtgcatgtagggctcggcctcctgcgaacagggcgtaggctgctcttcctcctctggggcctcggcaccagggccgttgggtgcctcttggaacaggatcttcttcatcttgcggtactgcaggttgtccagctcccgcacggcatccttggtcctctggatcaggtccatgatgactgtgggtggccgctcccggagcacaaagcggtgcttcaggagaacctctgaggttggtctgtcttgagggattttctgaagacaggagtcgacaaaattccggaagtactcagaccagtgtcctgactggagcacgggggattcgttctgtgcaatgtggtataaggcactcatcgcattcatgttaaagagcggtggtttccgttcagccagctcgatgcaggttatccccaaggaccagacgtccactttgccatcgtactgcccctcatccatggccaggatcacctcgggtgccatccagtatggggtgcccacgaaggagttggcaggtgccatgatggacgcagaaccaaagtcccctagcttcactaaccctggctctgacagcaggatgtttccagccttcacatccctatggatcatgttgtgggagtgcagatatgccaggccctgaagcgccccgtgggtcacagctgcgatctctacctcctgaaggggtttcttgtgcacttctagaaggtcagaagctgagcccaggcaatactccattaccagccaagccgtgtgctccctcaggtaacagccccggtactgaatggtgttgggatgccggagcttctgtaagaaccgcacctccttgatgatgtcttgccatttctcattggactgcttcccactgtaggacatcttcttgatggccaccacctcactattccggacatcccgggcaaagtatacggctccaaagctgccatggccaatttcccggaggtcagagaagagcttttctgggtcatccttgaagaagagctcagccacatctgggtccttcaggctcccggcccggcccccagctggcatggtggcccctgggggccctgagagtggggcctggcctggtaggggtcactatggtgccccagcgcctccgcttccgcctggggtcctccagcggctctgccaagcagggagaggggcaaggagacctttccccttgccacctcttcctcggctttcgcccttcctgaggggcgggcccgggaagcctcccctggaggggagggggtgacaacctaatctgacctcgcggtccagtcctccccctcgtcgagggcgacagctgccgaattccggatttctgattgtggggtctgaaccccgaatatctgaacgggatggagactgaatccgatatttgaacgcccggggaatgaaccccggatactggtgcacgcaggggcctgaacctgatatttgaaattctatgaaacagagacccaggtttagagaggttgggacccgagtcccggatatctggactatgaggactgttacccgggtatctgagaaaggaggaggggcaaagcctggaaatttgggacccaggggcctgagctgtaggtcttcggccaccgactgggggcccaccccgaggacgtccggccgcacggcccctctcacgccggggtccgagggtgacagcccccactcccgccccggcctcctccctctcccttctctcttccgagaatagctgaacgattgtagctaaggtgctgctgacggtccccgcgccctctctgcctctcctcttctccgtctcagcctctctccgcaccacagccccggtctcgtcccggtctccctctccctcttcctcccaattccaagatggag

SEQ ID NO: 18614 - RNA, 1334 nt, Homo sapiens
  source 1..1334: mol_type = other RNA
tgagtgtgtgtgtgtgagtgtgtaagaaccagatcagactggaaaaaactctctcccactgtgggttcactgtcaacaaaacatcaggccagccagtgtctaggctgtctcctcaatttccccaataatgtgcctcacattcctcacagaagcctcccaggcttcctgcacattctgtggcatttctcagtgacctagagggatctttaaaccgcaacgagcctaagtggctgaaaacctcaggaacgcctgtcagtgtcccagcaagttgagtctgagtgacacatctgagtttccactcctgagtgaggaaggcctcgctgctaacactcccctggggtgcgccgagaggaagcagtgggtgtgggtgggcgtccccaggctcagtccctgaacacacatgccgggcgggagacctgccctgaggctcggcagcccctcagtggggtctgctgctggactccaaatgtgaccgtttgccagaggtcagcatcccagggtggtcccctggctcagaaaaggtccgcttgtagctccgcccattggaccctcctcggtgccatttgcagatgtcaccattcagaatgtcctggatgtgctgcacgatcaggttgatggcaaccatattgtccactcctcgcgggatgatcacatcggcatacttctttgtcggcaggcagaactcctcgaaggccggcttcacgaaggtggtgtactgcgtcagaatctgctccaggtccctccctcggcgcacgtcccggagaactcttcgagacagcctgacgtcggagtcggtgtccacgaagaggcgcaggtggaacatgtcccggatctcctggctgtagaacaccaagatgccctcaaacagaaccacgtccgcagggtagaccaccgtggtctctggtaaccttgagtgtgtcacaaaatcataggtcggcacctccaccgttttgccctccacgatgttcttcagagtcctggatggtcaaaattgtactgtcctttcaaggccttggccttctgctctgccgtcaggaccttgtagaacctgtcctggctcaggatgaccaccttccgctgccgctgttccacctcgttctgtcccagcaactccatgatcttctcacacacggtcgacttcccgctggcagtgccgccgctcacccctatcaggaagggccgctggtgcggacggtcggcctccggcgcggggctctcgcagtcttcgcctcccgccgaagccatctcggcctccgctcccgcgcatcgggtccccgcgcccgccccttccccaggcccggcgcgcccgcccagcgccgaggtcggaggcaacc

SEQ ID NO: 18615 - RNA, 1335 nt, Homo sapiens
  source 1..1335: mol_type = other RNA
tgagtgtgtgtgtgtgagtgtgtaagaaccagatcagactggaaaaaactctctcccactgtgggttcactgtcaacaaaacatcaggccagccagtgtctaggctgtctcctcaatttccccaataatgtgcctcacattcctcacagaagcctcccaggcttcctgcacattctgtggcatttctcagtgacctagagggatctttaaaccgcaacgagcctaagtggctgaaaacctcaggaacgcctgtcagtgtcccagcaagttgagtctgagtgacacatctgagtttccactcctgagtgaggaaggcctcgctgctaacactcccctggggtgcgccgagaggaagcagtgggtgtgggtgggcgtccccaggctcagtccctgaacacacatgccgggcgggagacctgccctgaggctcggcagcccctcagtggggtctgctgctggactccaaatgtgaccgtttgccagaggtcagcatcccagggtggtcccctggctcagaaaaggtccgcttgtagctccgcccattggaccctcctcggtgccatttgcagatgtcaccattcagaatgtcctggatgtgctgcacgatcaggttgatggcaaccatattgtccactcctcgcgggatgatcacatcggcatacttctttgtcggcaggcagaactcctcgaaggccggcttcacgaaggtggtgtactgcgtcagaatctgctccaggtccctccctcggcgcacgtcccggagaactcttcgagacagcctgacgtcggagtcggtgtccacgaagaggcgcaggtggaacatgtcccggatctcctggctgtagaacaccaagatgccctcaaacagaaccacgtccgcagggtagaccaccgtggtctctggtaaccttgagtgtgtcacaaaatcataggtcggcacctccaccgttttgccctccacgatgttcttcagagtcctgtgcatcaaatcattatcaaaggcatctggatggtcaaaattgtactgtcctttcaaggccttggccttctgctctgccgtcaggaccttgtagaacctgtcctggctcaggatgaccaccttccgctgccgctgttccacctcgttctgtcccagcaactccatgatcttctcacacacggtcgaccctatcaggaagggccgctggtgcggacggtcggcctccggcgcggggctctcgcagtcttcgcctcccgccgaagccatctcggcctccgctcccgcgcatcgggtccccgcgcccgccccttccccaggcccggcgcgcccgcccagcgccgaggtcggaggcaacc

SEQ ID NO: 18616 - RNA, 1377 nt, Homo sapiens
  source 1..1377: mol_type = other RNA
tgagtgtgtgtgtgtgagtgtgtaagaaccagatcagactggaaaaaactctctcccactgtgggttcactgtcaacaaaacatcaggccagccagtgtctaggctgtctcctcaatttccccaataatgtgcctcacattcctcacagaagcctcccaggcttcctgcacattctgtggcatttctcagtgacctagagggatctttaaaccgcaacgagcctaagtggctgaaaacctcaggaacgcctgtcagtgtcccagcaagttgagtctgagtgacacatctgagtttccactcctgagtgaggaaggcctcgctgctaacactcccctggggtgcgccgagaggaagcagtgggtgtgggtgggcgtccccaggctcagtccctgaacacacatgccgggcgggagacctgccctgaggctcggcagcccctcagtggggtctgctgctggactccaaatgtgaccgtttgccagaggtcagcatcccagggtggtcccctggctcagaaaaggtccgcttgtagctccgcccattggaccctcctcggtgccatttgcagatgtcaccattcagaatgtcctggatgtgctgcacgatcaggttgatggcaaccatattgtccactcctcgcgggatgatcacatcggcatacttctttgtcggcaggcagaactcctcgaaggccggcttcacgaaggtggtgtactgcgtcagaatctgctccaggtccctccctcggcgcacgtcccggagaactcttcgagacagcctgacgtcggagtcggtgtccacgaagaggcgcaggtggaacatgtcccggatctcctggctgtagaacaccaagatgccctcaaacagaaccacgtccgcagggtagaccaccgtggtctctggtaaccttgagtgtgtcacaaaatcataggtcggcacctccaccgttttgccctccacgatgttcttcagagtcctgtgcatcaaatcattatcaaaggcatctggatggtcaaaattgtactgtcctttcaaggccttggccttctgctctgccgtcaggaccttgtagaacctgtcctggctcaggatgaccaccttccgctgccgctgttccacctcgttctgtcccagcaactccatgatcttctcacacacggtcgactggagacacagaagcgggattcccgcctggaaccgctcgtcccctatcaggaagggccgctggtgcggacggtcggcctccggcgcggggctctcgcagtcttcgcctcccgccgaagccatctcggcctccgctcccgcgcatcgggtccccgcgcccgccccttccccaggcccggcgcgcccgcccagcgccgaggtcggaggcaacc

SEQ ID NO: 18617 - RNA, 1338 nt, Homo sapiens
  source 1..1338: mol_type = other RNA
tgagtgtgtgtgtgtgagtgtgtaagaaccagatcagactggaaaaaactctctcccactgtgggttcactgtcaacaaaacatcaggccagccagtgtctaggctgtctcctcaatttccccaataatgtgcctcacattcctcacagaagcctcccaggcttcctgcacattctgtggcatttctcagtgacctagagggatctttaaaccgcaacgagcctaagtggctgaaaacctcaggaacgcctgtcagtgtcccagcaagttgagtctgagtgacacatctgagtttccactcctgagtgaggaaggcctcgctgctaacactcccctggggtgcgccgagaggaagcagtgggtgtgggtgggcgtccccaggctcagtccctgaacacacatgccgggcgggagacctgccctgaggctcggcagcccctcagtggggtctgctgctggactccaaatgtgaccgtttgccagaggtcagcatcccagggtggtcccctggctcagaaaaggtccgcttgtagctccgcccattggaccctcctcggtgccatttgcagatgtcaccattcagaatgtcctggatgtgctgcacgatcaggttgatggcaaccatattgtccactcctcgcgggatgatcacatcggcatacttctttgtcggcaggcagaactcctcgaaggccggcttcacgaaggtggtgtactgcgtcagaatctgctccaggtccctccctcggcgcacgtcccggagaactcttcgagacagcctgacgtcggagtcggtgtccacgaagaggcgcaggtggaacatgtcccggatctcctggctgtagaacaccaagatgccctcaaacagaaccacgtccgcagggtagaccaccgtggtctctggtaaccttgagtgtgtcacaaaatcataggtcggcacctccaccgttttgccctccacgatgttcttcagagtcctgtgcatcaaatcattatcaaaggcatctggatggtcaaaattgtactgtcctttcaaggccttggccttctgctctgccgtcaggaccttgtagaacctgtcctggctcaggatgaccaccttccgctgccgctgttccacctcgttctgtcccagcaactccatgatcttctcacacacggtcgactggagacacagaagcgggattcccgcctggaaccgctcgtccttcccgctggcagtgccgccgctcacccctatcaggaagggccgctggtgcggacggtcggcctccggcgcggggctctcgcagtcttcgcctcccgccgaagccatctcggcctccgctcccgcgcatc

SEQ ID NO: 18618 - RNA, 1362 nt, Homo sapiens
  source 1..1362: mol_type = other RNA
tgagtgtgtgtgtgtgagtgtgtaagaaccagatcagactggaaaaaactctctcccactgtgggttcactgtcaacaaaacatcaggccagccagtgtctaggctgtctcctcaatttccccaataatgtgcctcacattcctcacagaagcctcccaggcttcctgcacattctgtggcatttctcagtgacctagagggatctttaaaccgcaacgagcctaagtggctgaaaacctcaggaacgcctgtcagtgtcccagcaagttgagtctgagtgacacatctgagtttccactcctgagtgaggaaggcctcgctgctaacactcccctggggtgcgccgagaggaagcagtgggtgtgggtgggcgtccccaggctcagtccctgaacacacatgccgggcgggagacctgccctgaggctcggcagcccctcagtggggtctgctgctggactccaaatgtgaccgtttgccagaggtcagcatcccagggtggtcccctggctcagaaaaggtccgcttgtagctccgcccattggaccctcctcggtgccatttgcagatgtcaccattcagaatgtcctggatgtgctgcacgatcaggttgatggcaaccatattgtccactcctcgcgggatgatcacatcggcatacttctttgtcggcaggcagaactcctcgaaggccggcttcacgaaggtggtgtactgcgtcagaatctgctccaggtccctccctcggcgcacgtcccggagaactcttcgagacagcctgacgtcggagtcggtgtccacgaagaggcgcaggtggaacatgtcccggatctcctggctgtagaacaccaagatgccctcaaacagaaccacgtccgcagggtagaccaccgtggtctctggtaaccttgagtgtgtcacaaaatcataggtcggcacctccaccgttttgccctccacgatgttcttcagagtcctgtgcatcaaatcattatcaaaggcatctggatggtcaaaattgtactgtcctttcaaggccttggccttctgctctgccgtcaggaccttgtagaacctgtcctggctcaggatgaccaccttccgctgccgctgttccacctcgttctgtcccagcaactccatgatcttctcacacacggtcgacttcccgctggcagtgccgccgctcacccctatcaggaagggccgctggtgcggacggtcggcctccggcgcggggctctcgcagtcttcgcctcccgccgaagccatctcggcctccgctcccgcgcatcgggtccccgcgcccgccccttccccaggcccggcgcgcccgcccagcgccgaggtcggaggcaacc

SEQ ID NO: 18619 - RNA, 1293 nt, Homo sapiens
  source 1..1293: mol_type = other RNA
tgagtgtgtgtgtgtgagtgtgtaagaaccagatcagactggaaaaaactctctcccactgtgggttcactgtcaacaaaacatcaggccagccagtgtctaggctgtctcctcaatttccccaataatgtgcctcacattcctcacagaagcctcccaggcttcctgcacattctgtggcatttctcagtgacctagagggatctttaaaccgcaacgagcctaagtggctgaaaacctcaggaacgcctgtcagtgtcccagcaagttgagtctgagtgacacatctgagtttccactcctgagtgaggaaggcctcgctgctaacactcccctggggtgcgccgagaggaagcagtgggtgtgggtgggcgtccccaggctcagtccctgaacacacatgccgggcgggagacctgccctgaggctcggcagcccctcagtggggtctgctgctggactccaaatgtgaccgtttgccagaggtcagcatcccagggtggtcccctggctcagaaaaggtccgcttgtagctccgcccattggaccctcctcggtgccatttgcagatgtcaccattcagaatgtcctggatgtgctgcacgatcaggttgatggcaaccatattgtccactcctcgcgggatgatcacatcggcatacttctttgtcggcaggcagaactcctcgaaggccggcttcacgaaggtggtgtactgcgtcagaatctgctccaggtccctccctcggcgcacgtcccggagaactcttcgagacagcctgacgtcggagtcggtgtccacgaagaggcgcaggtggaacatgtcccggatctcctggcttgagtgtgtcacaaaatcataggtcggcacctccaccgttttgccctccacgatgttcttcagagtcctgtgcatcaaatcattatcaaaggcatctggatggtcaaaattgtactgtcctttcaaggccttggccttctgctctgccgtcaggaccttgtagaacctgtcctggctcaggatgaccaccttccgctgccgctgttccacctcgttctgtcccagcaactccatgatcttctcacacacggtcgacttcccgctggcagtgccgccgctcacccctatcaggaagggccgctggtgcggacggtcggcctccggcgcggggctctcgcagtcttcgcctcccgccgaagccatctcggcctccgctcccgcgcatcgggtccccgcgcccgccccttccccaggcccggcgcgcccgcccagcgccgaggtcggaggcaacc

SEQ ID NO: 18620 - RNA, 1267 nt, Homo sapiens
  source 1..1267: mol_type = other RNA
tgagtgtgtgtgtgtgagtgtgtaagaaccagatcagactggaaaaaactctctcccactgtgggttcactgtcaacaaaacatcaggccagccagtgtctaggctgtctcctcaatttccccaataatgtgcctcacattcctcacagaagcctcccaggcttcctgcacattctgtggcatttctcagtgacctagagggatctttaaaccgcaacgagcctaagtggctgaaaacctcaggaacgcctgtcagtgtcccagcaagttgagtctgagtgacacatctgagtttccactcctgagtgaggaaggcctcgctgctaacactcccctggggtgcgccgagaggaagcagtgggtgtgggtgggcgtccccaggctcagtccctgaacacacatgccgggcgggagacctgccctgaggctcggcagcccctcagtggggtctgctgctggactccaaatgtgaccgtttgccagaggtcagcatcccagggtggtcccctggctcagaaaaggtccgcttgtagctccgcccattggaccctcctcggtgccatttgcagatgtcaccattcagaatgtcctggatgtgctgcacgatcaggttgatggcaaccatattgtccactcctcgcgggatgatcacatcggcatacttctttgtctcttcgagacagcctgacgtcggagtcggtgtccacgaagaggcgcaggtggaacatgtcccggatctcctggctgtagaacaccaagatgccctcaaacagaaccacgtccgcagggtagaccaccgtggtctctggtaaccttgagtgtgtcacaaaatcataggtcggcacctccaccgttttgccctccacgatgttcttcagagtcctgtgcatcaaatcattatcaaaggcatctggatggtcaaaattgtactgtcctttcaaggccttggccttctgctctgccgtcaggaccttgtagaacctgtcctggctcaggatgaccaccttccgctgccgctgttccacctcgttctgtcccagcaactccatgatcttctcacacacggtcgacttcccgctggcagtgccgccgctcacccctatcaggaagggccgctggtgcggacggtcggcctccggcgcggggctctcgcagtcttcgcctcccgccgaagccatctcggcctccgctcccgcgcatcgggtccccgcgcccgccccttccccaggcccggcgcgcccgcccagcgccgaggtcggaggcaacc

SEQ ID NO: 18621 - RNA, 1867 nt, Homo sapiens
  source 1..1867: mol_type = other RNA
tgagtgtgtgtgtgtgagtgtgtaagaaccagatcagactggaaaaaactctctcccactgtgggttcactgtcaacaaaacatcaggccagccagtgtctaggctgtctcctcaatttccccaataatgtgcctcacattcctcacagaagcctcccaggcttcctgcacattctgtggcatttctcagtgacctagagggatctttaaaccgcaacgagcctaagtggctgaaaacctcaggaacgcctgtcagtgtcccagcaagttgagtctgagtgacacatctgagtttccactcctgagtgaggaaggcctcgctgctaacactcccctggggtgcgccgagaggaagcagtgggtgtgggtgggcgtccccaggctcagtccctgaacacacatgccgggcgggagacctgccctgaggctcggcagcccctcagtggggtctgctgctggactccaaatgtgaccgtttgccagaggtcagcatcccagggtggtcccctggctcagaaaaggtccgcttgtagctccgcccattggaccctcctcggtgccatttgcagatgtcaccattcagaatgtcctggatgtgctgcacgatcaggttgatggcaaccatattgtccactcctcgcgggatgatcacatcggcatacttctttgtctgtaaggcacaagggggggtgttcctgtgaggacttttccttcaaaggtgattttaagatgctcagaaacagatgcaacagcaggaggggcggccctggggtgctcagaggtgctggtgtcatcggcaaatgggggacacagactcagtcatcagccaggtgtgagaggccatgatccaagaagtgaggcagaaagtgcagctgaggcagccaaaagaaagtgcctcttccagtgtccccattccatcacagaagacagcccccttccagtgttcccactccattacaggagacagctggctacgctaacgactcaattcactgggccaagctaagtgtggcacttctacaaagtgtgacattgttcctctggaatcatgaagcttctgcaaataccctggcacagcaacaggacagccgccgccgtgcataattactgcaggcagagacgctgatggtaacttactccctcatccaaccactcattggctcaatgctgactctcattccctgtcagatgctctgctgcggcaggcagaactcctcgaaggccggcttcacgaaggtggtgtactgcgtcagaatctgctccaggtccctccctcggcgcacgtcccggagaactcttcgagacagcctgacgtcggagtcggtgtccacgaagaggcgcaggtggaacatgtcccggatctcctggctgtagaacaccaagatgccctcaaacagaaccacgtccgcagggtagaccaccgtggtctctggtaaccttgagtgtgtcacaaaatcataggtcggcacctccaccgttttgccctccacgatgttcttcagagtcctgtgcatcaaatcattatcaaaggcatctggatggtcaaaattgtactgtcctttcaaggccttggccttctgctctgccgtcaggaccttgtagaacctgtcctggctcaggatgaccaccttccgctgccgctgttccacctcgttctgtcccagcaactccatgatcttctcacacacggtcgactggagacacagaagcgggattcccgcctggaaccgctcgtccttcccgctggcagtgccgccgctcacccctatcaggaagggccgctggtgcggacggtcggcctccggcgcggggctctcgcagtcttcgcctcccgccgaagccatctcggcctccgctcccgcgcatc

SEQ ID NO: 18622 - RNA, 1463 nt, Homo sapiens
  source 1..1463: mol_type = other RNA
tgagtgtgtgtgtgtgagtgtgtaagaaccagatcagactggaaaaaactctctcccactgtgggttcactgtcaacaaaacatcaggccagccagtgtctaggctgtctcctcaatttccccaataatgtgcctcacattcctcacagaagcctcccaggcttcctgcacattctgtggcatttctcagtgacctagagggatctttaaaccgcaacgagcctaagtggctgaaaacctcaggaacgcctgtcagtgtcccagcaagttgagtctgagtgacacatctgagtttccactcctgagtgaggaaggcctcgctgctaacactcccctggggtgcgccgagaggaagcagtgggtgtgggtgggcgtccccaggctcagtccctgaacacacatgccgggcgggagacctgccctgaggctcggcagcccctcagtggggtctgctgctggactccaaatgtgaccgtttgccagaggtcagcatcccagggtggtcccctggctcagaaaaggtccgcttgtagctccgcccattggaccctcctcggtgccatttgcagatgtcaccattcagaatgtcctggatgtgctgcacgatcaggttgatggcaaccatattgtccactcctcgcgggatgatcacatcggcatacttctttgttccctcatccaaccactcattggctcaatgctgactctcattccctgtcagatgctctgcggcaggcagaactcctcgaaggccggcttcacgaaggtggtgtactgcgtcagaatctgctccaggtccctccctcggcgcacgtcccggagaactcttcgagacagcctgacgtcggagtcggtgtccacgaagaggcgcaggtggaacatgtcccggatctcctggctgtagaacaccaagatgccctcaaacagaaccacgtccgcagggtagaccaccgtggtctctggtaaccttgagtgtgtcacaaaatcataggtcggcacctccaccgttttgccctccacgatgttcttcagagtcctgtgcatcaaatcattatcaaaggcatctggatggtcaaaattgtactgtcctttcaaggccttggccttctgctctgccgtcaggaccttgtagaacctgtcctggctcaggatgaccaccttccgctgccgctgttccacctcgttctgtcccagcaactccatgatcttctcacacacggtcgactggagacacagaagcgggattcccgcctggaaccgctcgtccttcccgctggcagtgccgccgctcacccctatcaggaagggccgctggtgcggacggtcggcctccggcgcggggctctcgcagtcttcgcctcccgccgaagccatctcggcctccgctcccgcgcatcgggtccccgcgcccgccccttccccaggcccggcgcgcccgcccagcgccgaggtcggaggcaacc

SEQ ID NO: 18623 - RNA, 390 nt, Homo sapiens
  source 1..390: mol_type = other RNA
tgagtgtgtgtgtgtgagtgtgtacacctatgtgtgtactaggcagcccagcagtggactctagactagaccagacagcttgaccagcatcacttctctaggattgtcctttcctgttatccatgcagtaatctggttagggtgagttgggatttgacccacactgggcagctgggccagtcagtgtttccccagaaattggaatgaaggagtcaggtagctgtggatctctatcctagtggtgacgtttccttattcaaggaaagaaagcaaagtattaggaggtcccacaaggtgggggaggaatatgttaattgctgttgcagtttttttatggcagctaaatgatgctgaggggaacctcacaaataaaactgtcttgatagaaat

SEQ ID NO: 18624 - RNA, 3137 nt, Homo sapiens
  source 1..3137: mol_type = other RNA
tgagtgtgtgtgtgtgagtgtgtacatgtatacactagtgtgcgtatgatttgggggtatgaatgtgaatgtgtacatatgtatttatgatctgagtgtgtatgagtgtgaatgtgaacatgtgtgtgtgagtgggtatatgatttgggtgtgtgcaagtatgaatatgtattgtgtgcattaatgtgtatattttgggctgtgtatgagtgaatgtgaacatgtgtgcacgagtgtatatatgatctgggtgtgtatgagtgagcatgagtgaacatgtgtgcatgaatgtgagtatgatttgggtgtgtatgagtgtgaatgtgtgcacgagtgtatatatgatctgggtgtgtatgagtgagcatgaatgtgaacatgtgtgcatgaatatatgatttgggtgtgtatgagtgtgaatgtgtgcacgagtgtacaatcggtgtgtatgagtgagcatgaatgtgaacatgtgtgcacgagtgtatatatgatctgggtgtgtaggagtgagcatgaatgtgtatgcacaagtgtgtgtatgtgtgtatgatctgggtgtggagtgtgaatacgaacacgtatgcgcaagtatgtatatgatctgtgtatgtatgagtgagtgtgaatgtgtgcataagtgtgtgtatgatctgggtatgagtgattgtgaatgtgagcatgtgtgcacgagtgtgtatatgatctgggtgtgtgggagtgagcatgaatgtgtatgcacaagtgtgtgtttgtgtgtatgatctgggtgtgtaggagtgtgaatatgaacacgtgtgcacaaatgtgtatatgatccgagtatgtaggagtgagtgtgaatgtgaacatgtttgcacgtgtgtatatgatatgggtgcatgtgtgggtgtgtttgtgcaggtgcactgggagctttcagcattgagtctgtgtggcatccaggcttttctggatgatgtagaatcaaaccccataattaattccagtaacttagaaattttcacttatgaatactaaattctcctcacctagcaactgactgagcaggttgaacagcacccttcgccgttctcctgcagaaccccgtggaatggccctgctttctcagagtgctcctagcggtgatgagggagcccagctcattgcggttcgtgcagaaggctgtgtgccatctccgggactgcacggagaggcggaggctcaggcgtgggatctgagctcagtgggccctttaaggaccgctgcctcctttcctccctttggcattcagcatcgacttacgatggctcccagtcacagtccttgtcactgcctggcattacacagggccacagtcccttaactgaaacacttgggaccagttgcattttggaattcggaatgtttcttgatttcagagagagaagaggggatggactgttgggcagccctgattaaccctgcagcgtcttggctctagaggggcctacacggctgggagcgtctcggctctagagaggggcctgcactgccgggagcatctcagctctagagaggggcctgcactgctgggaagcctacacggctgggagcgtctcggctctagagccacagctgatgcatggcaacgatgagctctcctgcttagtgctgatgtgcctcagcccctaaccccactggtgtccagatgaggaacttgaggctcagagaagctaggtcaaggtgaacaccagtgttgagtttcagccccaggtctacctgatgctgactccacattgactgagttggcctggtccattgtgaggtcaggtagagccagggccgaggtggggatgccaaggtcccatgccgcaaagatgggtgggacggcacaggagccggtcatcatccccaaagacacagctccgaatacctcatcctgaaatcccaaagatcaaaatcccaaaagtataaatctggaaaaaataatgtcgatgttatttatttacatttttaaaaggtatgtatttgagaaacataaaaacacaacagaacatttcataggccactttacacaataaaataggcaatgataacaggtatttttgcataaacactgaggtaactaacgacggcggcatgggtgtagcagttataagaagacagaccataaagaaataagtcaaaagagaaacgtgtacacgtatatcgctacggttactaattgtgtgcacctagccctgtagctgtggtcatctgaaatatcagggattttagacttgagggattttgatctttagggatttcaacattccacattatggtgcttgggattgtgtctttcaggattatgatccaaactcagctgggcctcccctccctgccccaggattgtggagtgagaacgttgcagcaggagagaacaacgcagcaaagcacagcaggggaaccggaaatgctcaccttttgacagggtacttttagttctggggccttatcttaaggatattccaacatatacaaaaagattcatgcacagagatatttactttagtattatttaccataggaaaaaagttggaaacaatacattttatgttctgtaaaatgaaagaacagttaaataaatcatggctctaagacgactccagggctgtgtacggaagttcagggacagaatcagttgaggctgttccacctgagcctaagcttcctctgctgtatgtcgggaatcaggtgggggccaagcgagatcaccacagtgcaggccagtgtgcagggcacaggtgggcgccagggaggggacgccgcacagccccatgctctcgccaaaaacgtgcagcacaatttggaagaaaacatttccatcttcagggtcgtctgtgtctgttaaagtcgagtctagtttcgggtctcagagcacctccctaaagctgccgtaaaccaagaataaaattctaagccccacagccgatcgcgtggaccccgcctctgggccaaagggattccagagaaacctgaagaactagttcaggccgtgatgaggaggagtgggggctggacaggcctcattgtaccctcctccctttggaatttgggcagaactgaccagaaccaacattaaaacagagatctgaagactgacaaggctctctagcaataagataccaaattcc

SEQ ID NO: 18625 - RNA, 1785 nt, Homo sapiens
  source 1..1785: mol_type = other RNA
tgagtgtgtgtgtgtgagtgtgtacatgtgtgtgtgtctgtgggggattgggaccaaggaaacccaatgcagatctgtgagacagtagagacagtaggcgtcagctggccctcgaacttaccctctggtacccacagatgcgcacagctcacaaagctgtgtatggaaggtgtcagtggagcagggacagtcgttgggactaagaaactcagaagctagagacaggacagactctttctggcctcgtggtgagggagaggctttctggaggaggtcagccttcaggctggggctagggagatgccgagggaggggcaagcatgagctcaggaaggaggaaggcaatgtgcagttggggctagaggacagtgagagatggtgtgtaaagaccagagcctggtggggcaggacctcaggtgtcctgagaaagctgctcccctgcctgttggccttgcagttgtgttttcagcctggagtttcttcctgatgacatggccccaagagcaggagagtgcttcaaaggtcaacttcctgggctcattccaaagtgctttgggggaccttagccattgcctctgatgttcagaacctaagacggggttgtcctgggaaattgccagcgtgcctaaagttgatcaccaatccctggccagaggacaccaagagcccctgttattgtccatggaatgggaatgggctctgtcaacctgggccaagagtccggcctggagcagctttgtaggcagctttagcaacacggtgaaaagcaaaagcaggaggagttgaagctgtaaatgccagctgtatttttattggtcgtctgcaacttcaaagctttcacctctttaaaggaggcccacgcaggtatccagtcggctctccgagctcccggccttgatgccttattgattttcaatgtggcttgactcccaggtgggcagacttcaaactggtctgtatttttctgctgtcatgtttccatccttgttagtttccatctccagcaagatcctgggcatgtttgagggcagctttccttctttggctttctctcaatgttctggacagcatttcagacatccagggccgccaccgctggagttgtgtcttgtgtgattaatacccagctgtgccagatgctggcaagtgcaagagagaagatgcagccttgctctcaagggattcacacccatcggtccatctaagtgttttctcagtgtggtcactagggaaggtgtggccagcggtggagggtggggctggtcacttgatgccaccaccccctttaacacatgctcttcaggactgacctgaagctgccaagtgtttactgagctgttgtttgcccagtaccggggagaacaaacattcattcagtgcctactacaaatattcattaatacgttcattaagtgcctgtagtaggccaggcactgagctttgctgatatttactagtagctttatctaaatttcatgtaaattctatgccactctgtgaagcaggttattcttagctcccttttataaatgaccatgccggattgcaggggtttaataatttgcccaagcttacttcacaagcaaaaggctgagcagggtctgagctgctcttgcttgagcacaccaggctggactgggtgtctgtgtgtgttggggaggaaagggtacaggaagcttgtcatctcattggcacacaaatcctattcatgtggaataaatgagcaagatgaggcatatgtgtggcaataataacaaaagcaaacatttctggctgggtgcagtg

SEQ ID NO: 18626 - RNA, 614 nt, Homo sapiens
  source 1..614: mol_type = other RNA
tgagtgtgtgtgtgtgagtgtgtacatgtgtgtgtgtctgtgggggattgggaccaaggaaacccaatgcagatctgtgagacagtagagacagtaggcgtcagctggccctcgaacttaccctctggtacccacagatgcgcacagctcacaaagctgtgtatggaaggtgtcagtggagcagggacagtcgttgggactaagaaactcagaagctagagacaggacagactctttctggcctcgtggtgagggagaggctttctggaggaggtcagccttcaggctggggctagggagatgccgagggaggggcaagcatgagctcaggaaggaggaaggcaatgtgcagttggggctagaggacagtgagagatggtgtgtaaagaccagagcctggtggggcaggacctcaggtgtcctgagaaagctgctcccctgcctgttggccttgcagttgtgttttcagcctggagtttcttcctgatgacatggccccaagagcaggagagtgcttcaaaggtcaacttcctgggctcattcctcagccttggagtcacttcctctctcagcctgtggccagagcccagcatatggctctgccctgctccaag

SEQ ID NO: 18627 - RNA, 802 nt, Homo sapiens
  source 1..802: mol_type = other RNA
tgagtgtgtgtgtgtgagtgtgtacatgtgtgtgtgtctgtgggggattgggaccaaggaaacccaatgcagatctgtgagacagtagagacagtaggcgtcagctggccctcgaacttaccctctggtacccacagatgcgcacagctcacaaagctgtgtatggaaggtgtcagtggagcagggacagtcgttgggactaagaaactcagaagctagagacaggacagactctttctggcctcgtggtgagggagaggctttctggaggaggtcagccttcaggctggggctagggagatgccgagggaggggcaagcatgagctcaggaaggaggaaggcaatgtgcagttggggctagaggacagtgagagatggtgtgtaaagaccagagcctggtggggcaggacctcaggtgtcctgagaaagctgctcccctgcctgttggccttgcagttgtgttttcagcctggagtttcttcctgatgacatggccccaagagcaggagagtgcttcaaaggtcaacttcctgggctcattccttggcccctgctcagaggtgtgattctgggagaaggctgaccaggagcatgctgaagacagaggcaggactacctatgtgtgaaattccagcagcccagctctgctgatgacagaaatggccataataaaccaaggaggtcacaagtcaagcaaataatttggttgacaaataggagtataaacaagaccttgattaatgaatttcctaatagttctctgtttattgacattagctcagcttggtcattaagcctgac

SEQ ID NO: 18628 - RNA, 569 nt, Homo sapiens
  source 1..569: mol_type = other RNA
tgagtgtgtgtgtgtgagtgtgtatgtgtttcaagggagatttctgggatgatggtggtgtgaatgtgtatgtgtgtgagtgtgtgtgtttcaagggagatttctgagctgacagtggtgtcaatgtgtgagtgtgtgtgcatgtgagtgtgtgtgagtgtgagtgagtgagagcatgtgtgtgtgtgagagtgtgtgtgagagtgtgtgtttcaagggagattcctgggctcgggctcttggacattgggcagaaggctgtgtcctctcctttgaccagtctctgttgtgtttcttccctgagctcatcaagagcagcctcagccatcccaagagcccccagagctgtttgtgggcagctgagcctgtgcagcccagcctcacccttgtcacagtgggccctaccaccatgtttggcccccatgagccatggcattttcacagtcaccctgcatagaaccaaggctggtcaccctttcacagatggagacacaaggaggatgtagcagtagggtgagatcagatcacgaggcggcttttgcttgttttttgataagaaagttttattt

SEQ ID NO: 18629 - RNA, 1274 nt, Homo sapiens
  source 1..1274: mol_type = other RNA
tgagtgtgtgtgtgtgagtgtgtctgtgtgagtgtgtgtgtatgtgtgtgtaatatgggtttgttggttaaattctttacacaaatcccatcagaatatgtatgtagataatttctagaaatttcttttttcatctaatagattttgaggaggatcactctgtgacataggcaatattaatttcatttactcttcacaatgaccctatgaggtaggggctagtgttatcgtccgttatacagatggagaaactgtgacacagaaaggctaagtgagttgcacaagatcacacagcaagtaagtggcaaagctgggattgaaacctaggctatctggctttggagcacgaatgcttaatcactcttctgcaatacttggctttaaccactgcatcacagtctagcctagagatggaccatagtatatttataaccactgcccttttgatccatatgcaggctgtgtccagggttccactagtataaaaaaggatgcagagaagagctttgtgcagcagccagaggggttcttgcagggtagtggcccagctgtggagtatgcacaggttacattccaataaatactgttagattttattcccaagaggttgaaactttcccattcccagcagttgtgttagtgtgcccatcccccttggtgccatcgagggcatgcaggcagaaggaacagcctgtggagaggggcgtggatatggtttggggaatggcaagaagtccagtgaggctgaaggttgggttgtagttgctggttgcgaatgtaatctattttatgctctgcaaatttgatacacgataccacgatatttcattgtagtttttgtttgcatttccccaattaccaggaagcaatatcatctttttgtgtgtttatgagccatttgtgttttttcttctgtaaactttatgttcatatttttacactttcccaatgggatgtttatcttcttggtttgtaggtgctctagtattatgggatgttagtcttttgtcagttacatttgcacgaatattatctcatggcgtgttgctcttacaaactcaagtttttagatagtaacctggattgtcaaatgcgacaagacggtttctcagtcacagctgtggaatgtgtaacgagacaacctctctgaagggcagcttggtaatagataccaaatgtgctttaaatcgtgtacacttgctgatgctggtattctatatccatcctcctgttattcatgcttttgtgtcctcttttctcaaactgaatcagag

SEQ ID NO: 18630 - RNA, 3553 nt, Homo sapiens
  source 1..3553: mol_type = other RNA
tgagtgtgtgtgtgtgagtgtgtctgtgtgtgtgtgtgggggggggtgtgtgtcccgggtaaatatttgaatgaggttcctgggaggagaggacgtgtgtgtgcgcgttgggggggcgggggggcggtgaatgtatgtgtctttgtgcagggtttcggggtgcaaggaagcggtggatgttctcgcgtgtttattcctgcaggtggcttaactgtgcttgcgcgcgcgtggaaagctggggtcctttccgagtcaattatgcgaggtcatgtgcctggagaggtggtggcgctccctgaaggactcattgcagatggggcacttgagtttctcctctcgccgccgcttcaccaagggctccatcgcatactcctttttgtggtgcgacctcatatggtacaccaggtcggaggtcatgcggaaggaggcattgcacttggcgcaccagttctgcgcgggcagacacagcgaggtgaaggagggcggcagcagcgtgagcgccgagggcagctgcagctgcaagggccccgcggccgccgccgcagccgcggctgcagcggcagcggagctcttgggccagaaggcggtggcgtacaggaaggggctctgcttaggcaggccgccgccgccgctcggcagggacccgcaacctccgttcaggtccgcggccccctggagcttcaccgctagagggtccgcggcggcgggatagagtctggtggggcccacgccgtcggcggggtggcatggctcgagcgcgcccagcttctggcccagcaccagcggggacagctgcgagaaagagcgtgctggctgcgagaaggcgcttttgcgctcgtccgacgcggcgccctggcccccgcccgcgccgcctgcggccccggcgcccgttccgcccccaccgctggtgctgcccgcgctgcccagctgcggcaccgaagtgaaggcgctgcccctcgcaggactgccgccctcgagccggctgggcagcgggcccccaggccgcggggccagcagcttctcggcgcccaccggtgacgcggccgcgggcgtggaggagccgccgccgccgccagcgtcctggtcctcggaggcgactcccgcgccgtcggctgtcccctcctcctgcaggctggccgcgcgggcagccttcttcacctccacgaaggcgctgcgcttcgcctcgcccgtctcgggacttggcggcgcgaagaggcggccgttctcttccaggccgaagtagctgcccgaggctcggtactgctgcggtgtgcacaccagatcctccttggaggccgggaggggccgctctacgaagcggccccggccccctaccagaccagcgccaccgccgccctccgccgcctcctccgggaatttcctctttcctttgccgccgcccgtggcgatgccgtcgggactcagctccgcctcctggtggccgccgccgccgccgctgccgctaccgctgctgaggctctgggctggggagcagctgctgcctccccgggagttttccagctccctggccaggttgtggaagtctgtggatggcttcgcgctgctgccgccggcggcagcggatgggttgctgctttccggggagggggatgggtagtggtggagggggccggctttgcaaaacttgggacccgggcctaaaggtgcctcctgctgctgctgctgctggtctttgccaccgccgccgccgcccccgtggtccttggtgcccacgccgccgccttgttcgtcttggggacttatatcagcgctgtgaagtctcttggggcagcggaaacgcagatgcgccacataggggaactcaaactggaaacgttggctgcattccaggcatgtgtaaggggacgacccattcattttgttgtgggatctagaggggcagagcaagagtaactcagtcagttctttcccgtaccaaactagtaactcctcgtctttggcaatcctgcggagagagcggtagaacagctgtccgttttttatgtaggcttcaaggttctgctcttccttatctctggccgattggaccaaccgcagccacatgagaccttctgaggaaccatttgctgctgaggtgtctacccgaaagatatacggtactgttctcttgtcagtagacttgagagctatgaaagctatgctgtcatatagggaagtatggctcaggacacagggaccaaatatagcattctcagggatgtcgcaggtggtgtaaacgctggtaaaaatatctgtcagacattgttggacagccttggcatctccatcccagatgcctcgctggatgccagtatcctccatcacaggaataaggtcagtatagaatctcccaaataaggccacctggaaccgggaagatgcaatcgagtgtttccttttgcctattgtatcagtgtatttccatgtcaagaggtgttggtgttgccgccttttaggctcttccaaaatgattggagagggcctttccccgtttcactaggcacttggagaagctgtgacagagagctggacacccagcgcgtgcggaccccgtgcgtatttccccggagtccgcgttccgtgaaagggagaggggtgcggttagctccagggattctctagccctggagccaccgctgatttgcgcagctagttgcctgggggtgataaacgggcgtcgtctctcttcaggagcgccaacactaccaagcttcccccaagatgggctccggaaagcttttcacatccagcgggtggtggaggaggggatggagttgccgaggccgtctcgggagcctcgtttgtgcgctaagccacttagaggcgctgacttgcccctttagtgcagcagctgatgctaatgacttgaggtctttaacagcctgcaagttgactccttcaacggggctgcaacaccacgtcgctggggaatctcgggcttctttttcacagttcaattctctactccatgttagtttgatcctctcccagctttgagacccttctctggaactcagtggggtattgaggctttgacagcctggtgactgcagtcccaggaggccaggggaggattttgcttgttccactttagcaaggctctttggagtcctggcaaaaatacacatgtaggaaactgtagtgttattttggaagagtgggctggagagaggttgataaatgacaccccaggtggcttttatgacattatgaagtggaggcaagaataggcaaggattgtaacatatttgttctcttgaacttgctgagcgaaaagatgcttcccaggctgatttgatagtattttgccgccgcccctgacgattttccgggctccttgccggtgagtctgctccacttcaggaccgcatttttattgaagtgcaccctattatttcgctaatgagttgcgggtctcctcagtttcccttctgtccttgcacattcctctagcgaggctttttgtgaaattgtaggaaaacaagtctagtaggtcagagatcgcatttgctcgtgtaagggattaataaagctcttgtctgatgctgctttt

SEQ ID NO: 18631 - RNA, 3173 nt, Homo sapiens
  source 1..3173: mol_type = other RNA
tgagtgtgtgtgtgtgagtgtgtctgtgtgtgtgtgtgggggggggtgtgtgtcccgggtaaatatttgaatgaggttcctgggaggagaggacgtgtgtgtgcgcgttgggggggcgggggggcggtgaatgtatgtgtctttgtgcagggtttcggggtgcaaggaagcggtggatgttctcgcgtgtttattcctgcaggtggcttaactgtgcttgcgcgcgcgtggaaagctggggtcctttccgagtcaattatgcgaggtcatgtgcctggagaggtggtggcgctccctgaaggactcattgcagatggggcacttgagtttctcctctcgccgccgcttcaccaagggctccatcgcatactcctttttgtggtgcgacctcatatggtacaccaggtcggaggtcatgcggaaggaggcattgcacttggcgcaccagttctgcgcgggcagacacagcgaggtgaaggagggcggcagcagcgtgagcgccgagggcagctgcagctgcaagggccccgcggccgccgccgcagccgcggctgcagcggcagcggagctcttgggccagaaggcggtggcgtacaggaaggggctctgcttaggcaggccgccgccgccgctcggcagggacccgcaacctccgttcaggtccgcggccccctggagcttcaccgctagagggtccgcggcggcgggatagagtctggtggggcccacgccgtcggcggggtggcatggctcgagcgcgcccagcttctggcccagcaccagcggggacagctgcgagaaagagcgtgctggctgcgagaaggcgcttttgcgctcgtccgacgcggcgccctggcccccgcccgcgccgcctgcggccccggcgcccgttccgcccccaccgctggtgctgcccgcgctgcccagctgcggcaccgaagtgaaggcgctgcccctcgcaggactgccgccctcgagccggctgggcagcgggcccccaggccgcggggccagcagcttctcggcgcccaccggtgacgcggccgcgggcgtggaggagccgccgccgccgccagcgtcctggtcctcggaggcgactcccgcgccgtcggctgtcccctcctcctgcaggctggccgcgcgggcagccttcttcacctccacgaaggcgctgcgcttcgcctcgcccgtctcgggacttggcggcgcgaagaggcggccgttctcttccaggccgaagtagctgcccgaggctcggtactgctgcggtgtgcacaccagatcctccttggaggccgggaggggccgctctacgaagcggccccggccccctaccagaccagcgccaccgccgccctccgccgcctcctccgggaatttcctctttcctttgccgccgcccgtggcgatgccgtcgggactcagctccgcctcctggtggccgccgccgccgccgctgccgctaccgctgctgaggctctgggctggggagcagctgctgcctccccgggagttttccagctccctggccaggttgtggaagtctgtggatggcttcgcgctgctgccgccggcggcagcggatgggttgctgctttccggggagggggatgggtagtggtggagggggccggctttgcaaaacttgggacccgggcctaaaggtgcctcctgctgctgctgctgctggtctttgccaccgccgccgccgcccccgtggtccttggtgcccacgccgccgccttgttcgtcttggggacttatatcagcgctgtgaagtctcttggggcagcggaaacgcagatgcgccacataggggaactcaaactggaaacgttggctgcattccaggcatgtgtaaggggacgacccattcattttgttgtgggatctagaggggcagagcaagagtaactcagtcagttctttcccgtaccaaactagtaactcctcgtctttggcaatcctgcggagagagcggtagaacagctgtccgttttttatgtaggcttcaaggttctgctcttccttatctctggccgattggaccaaccgcagccacatgagaccttctgaggaaccatttgctgctgaggtgtctacccgaaagatatacggtactgttctcttgtcagtagacttgagagctatgaaagctatgctgtcatatagggaagtatggctcaggacacagggaccaaatatagcattctcagggatgtcgcaggtggtgtaaacgctggtaaaaatatctgtcagacattgttggacagccttggcatctccatcccagatgcctcgctggatgccagtatcctccatcacaggaataaggtcagtatagaatctcccaaataaggccacctggaaccgggaagatgcaatcgagtgtttccttttgcctattgtatcagtgtatttccatgtcaagaggtgttggtgttgccgccttttaggctcttccaaaatgattggagagggcctttccccgtttcactaggcacttggagaagctgtgacagagagctggacacccagcgcgtgcggaccccgtgcgtatttccccggagtccgcgttccgtgaaagggagaggggtgcggttagctccagggattctctagccctggagccaccgctgatttgcgcagctagttgcctgggggtgataaacgggcgtcgtctctcttcaggagcgccaacactaccaagcttcccccaagatgggctccggaaagcttttcacatccagcgggtggtggaggaggggatggagttgccgaggccgtctcgggagcctcgtttgtgcgctaagccacttagaggcgctgacttgcccctttagtgcagcagctgatgctaatgacttgaggtctttaacagcctgcaagttgactccttcaacggggctgcaacaccacgtcgctggggaatctcgggcttctttttcacagttcaattctctactccttgttccactttagcaaggctctttggagtcctggcaaaaatacacatgtaggaaactgtagtgttattttggaagagtgggctggagagaggttgataaatgacaccccaggtggcttttatgaccgctttccagcggaagggggcatctttgcggcagaggcagcgttccccggggcgggggcgggacgccggggcagagcca

SEQ ID NO: 18632 - RNA, 3041 nt, Homo sapiens
  source 1..3041: mol_type = other RNA
tgagtgtgtgtgtgtgagtgtgtctgtgtgtgtgtgtgggggggggtgtgtgtcccgggtaaatatttgaatgaggttcctgggaggagaggacgtgtgtgtgcgcgttgggggggcgggggggcggtgaatgtatgtgtctttgtgcagggtttcggggtgcaaggaagcggtggatgttctcgcgtgtttattcctgcaggtggcttaactgtgcttgcgcgcgcgtggaaagctggggtcctttccgagtcaattatgcgaggtcatgtgcctggagaggtggtggcgctccctgaaggactcattgcagatggggcacttgagtttctcctctcgccgccgcttcaccaagggctccatcgcatactcctttttgtggtgcgacctcatatggtacaccaggtcggaggtcatgcggaaggaggcattgcacttggcgcaccagttctgcgcgggcagacacagcgaggtgaaggagggcggcagcagcgtgagcgccgagggcagctgcagctgcaagggccccgcggccgccgccgcagccgcggctgcagcggcagcggagctcttgggccagaaggcggtggcgtacaggaaggggctctgcttaggcaggccgccgccgccgctcggcagggacccgcaacctccgttcaggtccgcggccccctggagcttcaccgctagagggtccgcggcggcgggatagagtctggtggggcccacgccgtcggcggggtggcatggctcgagcgcgcccagcttctggcccagcaccagcggggacagctgcgagaaagagcgtgctggctgcgagaaggcgcttttgcgctcgtccgacgcggcgccctggcccccgcccgcgccgcctgcggccccggcgcccgttccgcccccaccgctggtgctgcccgcgctgcccagctgcggcaccgaagtgaaggcgctgcccctcgcaggactgccgccctcgagccggctgggcagcgggcccccaggccgcggggccagcagcttctcggcgcccaccggtgacgcggccgcgggcgtggaggagccgccgccgccgccagcgtcctggtcctcggaggcgactcccgcgccgtcggctgtcccctcctcctgcaggctggccgcgcgggcagccttcttcacctccacgaaggcgctgcgcttcgcctcgcccgtctcgggacttggcggcgcgaagaggcggccgttctcttccaggccgaagtagctgcccgaggctcggtactgctgcggtgtgcacaccagatcctccttggaggccgggaggggccgctctacgaagcggccccggccccctaccagaccagcgccaccgccgccctccgccgcctcctccgggaatttcctctttcctttgccgccgcccgtggcgatgccgtcgggactcagctccgcctcctggtggccgccgccgccgccgctgccgctaccgctgctgaggctctgggctggggagcagctgctgcctccccgggagttttccagctccctggccaggttgtggaagtctgtggatggcttcgcgctgctgccgccggcggcagcggatgggttgctgctttccggggagggggatgggtagtggtggagggggccggctttgcaaaacttgggacccgggcctaaaggtgcctcctgctgctgctgctgctggtctttgccaccgccgccgccgcccccgtggtccttggtgcccacgccgccgccttgttcgtcttggggacttatatcagcgctgtgaagtctcttggggcagcggaaacgcagatgcgccacataggggaactcaaactggaaacgttggctgcattccaggcatgtgtaaggggacgacccattcattttgttgtgggatctagaggggcagagcaagagtaactcagtcagttctttcccgtaccaaactagtaactcctcgtctttggcaatcctgcggagagagcggtagaacagctgtccgttttttatgtaggcttcaaggttctgctcttccttatctctggccgattggaccaaccgcagccacatgagaccttctgaggaaccatttgctgctgaggtgtctacccgaaagatatacggtactgttctcttgtcagtagacttgagagctatgaaagctatgctgtcatatagggaagtatggctcaggacacagggaccaaatatagcattctcagggatgtcgcaggtggtgtaaacgctggtaaaaatatctgtcagacattgttggacagccttggcatctccatcccagatgcctcgctggatgccagtatcctccatcacaggaataaggtcagtatagaatctcccaaataaggccacctggaaccgggaagatgcaatcgagtgtttccttttgcctattgtatcagtgtatttccatgtcaagaggtgttggtgttgccgccttttaggctcttccaagatgggctccggaaagcttttcacatccagcgggtggtggaggaggggatggagttgccgaggccgtctcgggagcctcgtttgtgcgctaagccacttagaggcgctgacttgcccctttagtgcagcagctgatgctaatgacttgaggtctttaacagcctgcaagttgactccttcaacggggctgcaacaccacgtcgctggggaatctcgggcttctttttcacagttcaattctctactccatgttagtttgatcctctcccagctttgagacccttctctggaactcagtggggtattgaggctttgacagcctggtgactgcagtcccaggaggccaggggaggattttgcttgttccactttagcaaggctctttggagtcctggcaaaaatacacatgtaggaaactgtagtgttattttggaagagtgggctggagagaggttgataaatgacaccccaggtggcttttatgacattatgaagtggaggcaagaataggcaaggattgtaacatatttgttctcttgaacttgctgagcgaaaagatgcttcccaggctgatt

SEQ ID NO: 18633 - RNA, 2585 nt, Homo sapiens
  source 1..2585: mol_type = other RNA
tgagtgtgtgtgtgtgagtgtgtctgtgtgtgtgtgtgggggggggtgtgtgtcccgggtaaatatttgaatgaggttcctgggaggagaggacgtgtgtgtgcgcgttgggggggcgggggggcggtgaatgtatgtgtctttgtgcagggtttcggggtgcaaggaagcggtggatgttctcgcgtgtttattcctgcaggtggcttaactgtgcttgcgcgcgcgtggaaagctggggtcctttccgagtcaattatgcgaggtcatgtgcctggagaggtggtggcgctccctgaaggactcattgcagatggggcacttgagtttctcctctcgccgccgcttcaccaagggctccatcgcatactcctttttgtggtgcgacctcatatggtacaccaggtcggaggtcatgcggaaggaggcattgcacttggcgcaccagttctgcgcgggcagacacagcgaggtgaaggagggcggcagcagcgtgagcgccgagggcagctgcagctgcaagggccccgcggccgccgccgcagccgcggctgcagcggcagcggagctcttgggccagaaggcggtggcgtacaggaaggggctctgcttaggcaggccgccgccgccgctcggcagggacccgcaacctccgttcaggtccgcggccccctggagcttcaccgctagagggtccgcggcggcgggatagagtctggtggggcccacgccgtcggcggggtggcatggctcgagcgcgcccagcttctggcccagcaccagcggggacagctgcgagaaagagcgtgctggctgcgagaaggcgcttttgcgctcgtccgacgcggcgccctggcccccgcccgcgccgcctgcggccccggcgcccgttccgcccccaccgctggtgctgcccgcgctgcccagctgcggcaccgaagtgaaggcgctgcccctcgcaggactgccgccctcgagccggctgggcagcgggcccccaggccgcggggccagcagcttctcggcgcccaccggtgacgcggccgcgggcgtggaggagccgccgccgccgccagcgtcctggtcctcggaggcgactcccgcgccgtcggctgtcccctcctcctgcaggctggccgcgcgggcagccttcttcacctccacgaaggcgctgcgcttcgcctcgcccgtctcgggacttggcggcgcgaagaggcggccgttctcttccaggccgaagtagctgcccgaggctcggtactgctgcggtgtgcacaccagatcctccttggaggccgggaggggccgctctacgaagcggccccggccccctaccagaccagcgccaccgccgccctccgccgcctcctccgggaatttcctctttcctttgccgccgcccgtggcgatgccgtcgggactcagctccgcctcctggtggccgccgccgccgccgctgccgctaccgctgctgaggctctgggctggggagcagctgctgcctccccgggagttttccagctccctggccaggttgtggaagtctgtggatggcttcgcgctgctgccgccggcggcagcggatgggttgctgctttccggggagggggatgggtagtggtggagggggccggctttgcaaaacttgggacccgggcctaaaggtgcctcctgctgctgctgctgctggtctttgccaccgccgccgccgcccccgtggtccttggtgcccacgccgccgccttgttcgtcttggggacttatatcagcgctgtgaagtctcttggggcagcggaaacgcagatgcgccacataggggaactcaaactggaaacgttggctgcattccaggcatgtgtaaggggacgacccattcattttgttgtgggatctagaggggcagagcaagagtaactcagtcagttctttcccgtaccaaactagtaactcctcgtctttggcaatcctgcggagagagcggtagaacagctgtccgttttttatgtaggcttcaaggttctgctcttccttatctctggccgattggaccaaccgcagccacatgagaccttctgaggaaccatttgctgctgaggtgtctacccgaaagatatacggtactgttctcttgtcagtagacttgagagctatgaaagctatgctgtcatatagggaagtatggctcaggacacagggaccaaatatagcattctcagggatgtcgcaggtggtgtaaacgctggtaaaaatatctgtcagacattgttggacagccttggcatctccatcccagatgcctcgctggatgccagtatcctccatcacaggaataaggtcagtatagaatctcccaaataaggccacctggaaccgggaagatgcaatcgagtgtttccttttgcctattgtatcagtgtatttccatgtcaagaggtgttggtgttgccgccttttaggctcttcctgaagagataagagagagatggagagatggggagaaaaagattgggggggtggagggagggagggagggagagagacggagaaacggagagagttgtacagatggacccgatgcagtgact

SEQ ID NO: 18634 - RNA, 3145 nt, Homo sapiens
  source 1..3145: mol_type = other RNA
tgagtgtgtgtgtgtgagtgtgtctgtgtgtgtgtgtgggggggggtgtgtgtcccgggtaaatatttgaatgaggttcctgggaggagaggacgtgtgtgtgcgcgttgggggggcgggggggcggtgaatgtatgtgtctttgtgcagggtttcggggtgcaaggaagcggtggatgttctcgcgtgtttattcctgcaggtggcttaactgtgcttgcgcgcgcgtggaaagctggggtcctttccgagtcaattatgcgaggtcatgtgcctggagaggtggtggcgctccctgaaggactcattgcagatggggcacttgagtttctcctctcgccgccgcttcaccaagggctccatcgcatactcctttttgtggtgcgacctcatatggtacaccaggtcggaggtcatgcggaaggaggcattgcacttggcgcaccagttctgcgcgggcagacacagcgaggtgaaggagggcggcagcagcgtgagcgccgagggcagctgcagctgcaagggccccgcggccgccgccgcagccgcggctgcagcggcagcggagctcttgggccagaaggcggtggcgtacaggaaggggctctgcttaggcaggccgccgccgccgctcggcagggacccgcaacctccgttcaggtccgcggccccctggagcttcaccgctagagggtccgcggcggcgggatagagtctggtggggcccacgccgtcggcggggtggcatggctcgagcgcgcccagcttctggcccagcaccagcggggacagctgcgagaaagagcgtgctggctgcgagaaggcgcttttgcgctcgtccgacgcggcgccctggcccccgcccgcgccgcctgcggccccggcgcccgttccgcccccaccgctggtgctgcccgcgctgcccagctgcggcaccgaagtgaaggcgctgcccctcgcaggactgccgccctcgagccggctgggcagcgggcccccaggccgcggggccagcagcttctcggcgcccaccggtgacgcggccgcgggcgtggaggagccgccgccgccgccagcgtcctggtcctcggaggcgactcccgcgccgtcggctgtcccctcctcctgcaggctggccgcgcgggcagccttcttcacctccacgaaggcgctgcgcttcgcctcgcccgtctcgggacttggcggcgcgaagaggcggccgttctcttccaggccgaagtagctgcccgaggctcggtactgctgcggtgtgcacaccagatcctccttggaggccgggaggggccgctctacgaagcggccccggccccctaccagaccagcgccaccgccgccctccgccgcctcctccgggaatttcctctttcctttgccgccgcccgtggcgatgccgtcgggactcagctccgcctcctggtggccgccgccgccgccgctgccgctaccgctgctgaggctctgggctggggagcagctgctgcctccccgggagttttccagctccctggccaggttgtggaagtctgtggatggcttcgcgctgctgccgccggcggcagcggatgggttgctgctttccggggagggggatgggtagtggtggagggggccggctttgcaaaacttgggacccgggcctaaaggtgcctcctgctgctgctgctgctggtctttgccaccgccgccgccgcccccgtggtccttggtgcccacgccgccgccttgttcgtcttggggacttatatcagcgctgtgaagtctcttggggcagcggaaacgcagatgcgccacataggggaactcaaactggaaacgttggctgcattccaggcatgtgtaaggggacgaccctgcattcattttgttgtgggatctagaggggcagagcaagagtaactcagtcagttctttcccgtaccaaactagtaactcctcgtctttggcaatcctgcggagagagcggtagaacagctgtccgttttttatgtaggcttcaaggttctgctcttccttatctctggccgattggaccaaccgcagccacatgagaccttctgaggaaccatttgctgctgaggtgtctacccgaaagatatacggtactgttctcttgtcagtagacttgagagctatgaaagctatgctgtcatatagggaagtatggctcaggacacagggaccaaatatagcattctcagggatgtcgcaggtggtgtaaacgctggtaaaaatatctgtcagacattgttggacagccttggcatctccatcccagatgcctcgctggatgccagtatcctccatcacaggaataaggtcagtatagaatctcccaaataaggccacctggaaccgggaagatgcaatcgagtgtttccttttgcctattgtatcagtgtatttccatgtcaagaggtgttggtgttgccgccttttaggctcttccaaaatgattggagagggcctttccccgtttcactaggcacttggagaagctgtgacagagagctggacacccagcgcgtgcggaccccgtgcgtatttccccggagtccgcgttccgtgaaagggagaggggtgcggttagctccagggattctctagccctggagccaccgctgatttgcgcagctagttgcctgggggtgataaacgggcgtcgtctctcttcaggagcgccaacactaccaagcttcccccaagatgggctccggaaagcttttcacatccagcgggtggtggaggaggggatggagttgccgaggccgtctcgggagcctcgtttgtgcgctaagccacttagaggcgctgacttgcccctttagtgcagcagctgatgctaatgacttgaggtctttaacagcctgcaagttgactccttcaacggggctgcaacaccacgtcgctggggaatctcgggcttctttttcacagttcaattctctactcctggggactgtggggctccttccccgggagcgcagctactgcgggcccctcggcggccgctctcccaccccaatcggagcctgccgaggagcccgtccgcctcgcgaaatggccccggtctctgctgcagcagctgggagggagggagcgaccgccggctgctgccgggcggcgt

SEQ ID NO: 18635 - RNA, 3372 nt, Homo sapiens
  source 1..3372: mol_type = other RNA
tgagtgtgtgtgtgtgagtgtgtctgtgtgtgtgtgtgggggggggtgtgtgtcccgggtaaatatttgaatgaggttcctgggaggagaggacgtgtgtgtgcgcgttgggggggcgggggggcggtgaatgtatgtgtctttgtgcagggtttcggggtgcaaggaagcggtggatgttctcgcgtgtttattcctgcaggtggcttaactgtgcttgcgcgcgcgtggaaagctggggtcctttccgagtcaattatgcgaggtcatgtgcctggagaggtggtggcgctccctgaaggactcattgcagatggggcacttgagtttctcctctcgccgccgcttcaccaagggctccatcgcatactcctttttgtggtgcgacctcatatggtacaccaggtcggaggtcatgcggaaggaggcattgcacttggcgcaccagttctgcgcgggcagacacagcgaggtgaaggagggcggcagcagcgtgagcgccgagggcagctgcagctgcaagggccccgcggccgccgccgcagccgcggctgcagcggcagcggagctcttgggccagaaggcggtggcgtacaggaaggggctctgcttaggcaggccgccgccgccgctcggcagggacccgcaacctccgttcaggtccgcggccccctggagcttcaccgctagagggtccgcggcggcgggatagagtctggtggggcccacgccgtcggcggggtggcatggctcgagcgcgcccagcttctggcccagcaccagcggggacagctgcgagaaagagcgtgctggctgcgagaaggcgcttttgcgctcgtccgacgcggcgccctggcccccgcccgcgccgcctgcggccccggcgcccgttccgcccccaccgctggtgctgcccgcgctgcccagctgcggcaccgaagtgaaggcgctgcccctcgcaggactgccgccctcgagccggctgggcagcgggcccccaggccgcggggccagcagcttctcggcgcccaccggtgacgcggccgcgggcgtggaggagccgccgccgccgccagcgtcctggtcctcggaggcgactcccgcgccgtcggctgtcccctcctcctgcaggctggccgcgcgggcagccttcttcacctccacgaaggcgctgcgcttcgcctcgcccgtctcgggacttggcggcgcgaagaggcggccgttctcttccaggccgaagtagctgcccgaggctcggtactgctgcggtgtgcacaccagatcctccttggaggccgggaggggccgctctacgaagcggccccggccccctaccagaccagcgccaccgccgccctccgccgcctcctccgggaatttcctctttcctttgccgccgcccgtggcgatgccgtcgggactcagctccgcctcctggtggccgccgccgccgccgctgccgctaccgctgctgaggctctgggctggggagcagctgctgcctccccgggagttttccagctccctggccaggttgtggaagtctgtggatggcttcgcgctgctgccgccggcggcagcggatgggttgctgctttccggggagggggatgggtagtggtggagggggccggctttgcaaaacttgggacccgggcctaaaggtgcctcctgctgctgctgctgctggtctttgccaccgccgccgccgcccccgtggtccttggtgcccacgccgccgccttgttcgtcttggggacttatatcagcgctgtgaagtctcttggggcagcggaaacgcagatgcgccacataggggaactcaaactggaaacgttggctgcattccaggcatgtgtaaggggacgaccctgcattcattttgttgtgggatctagaggggcagagcaagagtaactcagtcagttctttcccgtaccaaactagtaactcctcgtctttggcaatcctgcggagagagcggtagaacagctgtccgttttttatgtaggcttcaaggttctgctcttccttatctctggccgattggaccaaccgcagccacatgagaccttctgaggaaccatttgctgctgaggtgtctacccgaaagatatacggtactgttctcttgtcagtagacttgagagctatgaaagctatgctgtcatatagggaagtatggctcaggacacagggaccaaatatagcattctcagggatgtcgcaggtggtgtaaacgctggtaaaaatatctgtcagacattgttggacagccttggcatctccatcccagatgcctcgctggatgccagtatcctccatcacaggaataaggtcagtatagaatctcccaaataaggccacctggaaccgggaagatgcaatcgagtgtttccttttgcctattgtatcagtgtatttccatgtcaagaggtgttggtgttgccgccttttaggctcttccaaaatgattggagagggcctttccccgtttcactaggcacttggagaagctgtgacagagagctggacacccagcgcgtgcggaccccgtgcgtatttccccggagtccgcgttccgtgaaagggagaggggtgcggttagctccagggattctctagccctggagccaccgctgatttgcgcagctagttgcctgggggtgataaacgggcgtcgtctctcttcaggagcgccaacactaccaagcttcccccaagatgggctccggaaagcttttcacatccagcgggtggtggaggaggggatggagttgccgaggccgtctcgggagcctcgtttgtgcgctaagccacttagaggcgctgacttgcccctttagtgcagcagctgatgctaatgacttgaggtctttaacagcctgcaagttgactccttcaacggggctgcaacaccacgtcgctggggaatctcgggcttctttttcacagttcaattctctactccttgttccactttagcaaggctctttggagtcctggcaaaaatacacatgtaggaaactgtagtgttattttggaagagtgggctggagagaggttgataaatgacaccccaggtggcttttatgacattatgaagtggaggcaagaataggcaaggattgtaacatatttgttctcttgaacttgctgagcgaaaagatgcttcccaggctgatttgatagtatctggggactgtggggctccttccccgggagcgcagctactgcgggcccctcggcggccgctctcccaccccaatcggagcctgccgaggagcccgtccgcctcgcgaaatggccccggtctctgctgcagcagctgggagggagggagcgaccgccggctgctgccgggcggcgtct

SEQ ID NO: 18636 - RNA, 3197 nt, Homo sapiens
  source 1..3197: mol_type = other RNA
tgagtgtgtgtgtgtgagtgtgtctgtgtgtgtgtgtgggggggggtgtgtgtcccgggtaaatatttgaatgaggttcctgggaggagaggacgtgtgtgtgcgcgttgggggggcgggggggcggtgaatgtatgtgtctttgtgcagggtttcggggtgcaaggaagcggtggatgttctcgcgtgtttattcctgcaggtggcttaactgtgcttgcgcgcgcgtggaaagctggggtcctttccgagtcaattatgcgaggtcatgtgcctggagaggtggtggcgctccctgaaggactcattgcagatggggcacttgagtttctcctctcgccgccgcttcaccaagggctccatcgcatactcctttttgtggtgcgacctcatatggtacaccaggtcggaggtcatgcggaaggaggcattgcacttggcgcaccagttctgcgcgggcagacacagcgaggtgaaggagggcggcagcagcgtgagcgccgagggcagctgcagctgcaagggccccgcggccgccgccgcagccgcggctgcagcggcagcggagctcttgggccagaaggcggtggcgtacaggaaggggctctgcttaggcaggccgccgccgccgctcggcagggacccgcaacctccgttcaggtccgcggccccctggagcttcaccgctagagggtccgcggcggcgggatagagtctggtggggcccacgccgtcggcggggtggcatggctcgagcgcgcccagcttctggcccagcaccagcggggacagctgcgagaaagagcgtgctggctgcgagaaggcgcttttgcgctcgtccgacgcggcgccctggcccccgcccgcgccgcctgcggccccggcgcccgttccgcccccaccgctggtgctgcccgcgctgcccagctgcggcaccgaagtgaaggcgctgcccctcgcaggactgccgccctcgagccggctgggcagcgggcccccaggccgcggggccagcagcttctcggcgcccaccggtgacgcggccgcgggcgtggaggagccgccgccgccgccagcgtcctggtcctcggaggcgactcccgcgccgtcggctgtcccctcctcctgcaggctggccgcgcgggcagccttcttcacctccacgaaggcgctgcgcttcgcctcgcccgtctcgggacttggcggcgcgaagaggcggccgttctcttccaggccgaagtagctgcccgaggctcggtactgctgcggtgtgcacaccagatcctccttggaggccgggaggggccgctctacgaagcggccccggccccctaccagaccagcgccaccgccgccctccgccgcctcctccgggaatttcctctttcctttgccgccgcccgtggcgatgccgtcgggactcagctccgcctcctggtggccgccgccgccgccgctgccgctaccgctgctgaggctctgggctggggagcagctgctgcctccccgggagttttccagctccctggccaggttgtggaagtctgtggatggcttcgcgctgctgccgccggcggcagcggatgggttgctgctttccggggagggggatgggtagtggtggagggggccggctttgcaaaacttgggacccgggcctaaaggtgcctcctgctgctgctgctgctggtctttgccaccgccgccgccgcccccgtggtccttggtgcccacgccgccgccttgttcgtcttggggacttatatcagcgctgtgaagtctcttggggcagcggaaacgcagatgcgccacataggggaactcaaactggaaacgttggctgcattccaggcatgtgtaaggggacgaccctgcattcattttgttgtgggatctagaggggcagagcaagagtaactcagtcagttctttcccgtaccaaactagtaactcctcgtctttggcaatcctgcggagagagcggtagaacagctgtccgttttttatgtaggcttcaaggttctgctcttccttatctctggccgattggaccaaccgcagccacatgagaccttctgaggaaccatttgctgctgaggtgtctacccgaaagatatacggtactgttctcttgtcagtagacttgagagctatgaaagctatgctgtcatatagggaagtatggctcaggacacagggaccaaatatagcattctcagggatgtcgcaggtggtgtaaacgctggtaaaaatatctgtcagacattgttggacagccttggcatctccatcccagatgcctcgctggatgccagtatcctccatcacaggaataaggtcagtatagaatctcccaaataaggccacctggaaccgggaagatgcaatcgagtgtttccttttgcctattgtatcagtgtatttccatgtcaagaggtgttggtgttgccgccttttaggctcttccaagatgggctccggaaagcttttcacatccagcgggtggtggaggaggggatggagttgccgaggccgtctcgggagcctcgtttgtgcgctaagccacttagaggcgctgacttgcccctttagtgcagcagctgatgctaatgacttgaggtctttaacagcctgcaagttgactccttcaacggggctgcaacaccacgtcgctggggaatctcgggcttctttttcacagttcaattctctactcattatgaagtggaggcaagaataggcaaggattgtaacatatttgttctcttgaacttgctgagcgaaaagatgcttcccaggctgatttgatagtatcccccaatcaaacagtcgccgtgccccgtcccccgaaaagaatgacttcaacctctgagagctgccattctcagggctgctttcgcgagcacccagggaggcacctatggagaggagccagagccagaacctgagcgtgaaacacatccatcccctccacactaccttccggcgggcgacaaaccctccccccgccagtgatcagaaaagaaaaggaaaagtaccggggtgcaagcggggagggagggggaagtaagaaaacaagcgcagagagaaagagagaggaagagaggacgagggaggggggagagagagagagaagcaaaaaggaaacgagagaggagtacagttagaactgagaaaaatggggaaggggtggtcgc

SEQ ID NO: 18637 - RNA, 3452 nt, Homo sapiens
  source 1..3452: mol_type = other RNA
tgagtgtgtgtgtgtgagtgtgtctgtgtgtgtgtgtgggggggggtgtgtgtcccgggtaaatatttgaatgaggttcctgggaggagaggacgtgtgtgtgcgcgttgggggggcgggggggcggtgaatgtatgtgtctttgtgcagggtttcggggtgcaaggaagcggtggatgttctcgcgtgtttattcctgcaggtggcttaactgtgcttgcgcgcgcgtggaaagctggggtcctttccgagtcaattatgcgaggtcatgtgcctggagaggtggtggcgctccctgaaggactcattgcagatggggcacttgagtttctcctctcgccgccgcttcaccaagggctccatcgcatactcctttttgtggtgcgacctcatatggtacaccaggtcggaggtcatgcggaaggaggcattgcacttggcgcaccagttctgcgcgggcagacacagcgaggtgaaggagggcggcagcagcgtgagcgccgagggcagctgcagctgcaagggccccgcggccgccgccgcagccgcggctgcagcggcagcggagctcttgggccagaaggcggtggcgtacaggaaggggctctgcttaggcaggccgccgccgccgctcggcagggacccgcaacctccgttcaggtccgcggccccctggagcttcaccgctagagggtccgcggcggcgggatagagtctggtggggcccacgccgtcggcggggtggcatggctcgagcgcgcccagcttctggcccagcaccagcggggacagctgcgagaaagagcgtgctggctgcgagaaggcgcttttgcgctcgtccgacgcggcgccctggcccccgcccgcgccgcctgcggccccggcgcccgttccgcccccaccgctggtgctgcccgcgctgcccagctgcggcaccgaagtgaaggcgctgcccctcgcaggactgccgccctcgagccggctgggcagcgggcccccaggccgcggggccagcagcttctcggcgcccaccggtgacgcggccgcgggcgtggaggagccgccgccgccgccagcgtcctggtcctcggaggcgactcccgcgccgtcggctgtcccctcctcctgcaggctggccgcgcgggcagccttcttcacctccacgaaggcgctgcgcttcgcctcgcccgtctcgggacttggcggcgcgaagaggcggccgttctcttccaggccgaagtagctgcccgaggctcggtactgctgcggtgtgcacaccagatcctccttggaggccgggaggggccgctctacgaagcggccccggccccctaccagaccagcgccaccgccgccctccgccgcctcctccgggaatttcctctttcctttgccgccgcccgtggcgatgccgtcgggactcagctccgcctcctggtggccgccgccgccgccgctgccgctaccgctgctgaggctctgggctggggagcagctgctgcctccccgggagttttccagctccctggccaggttgtggaagtctgtggatggcttcgcgctgctgccgccggcggcagcggatgggttgctgctttccggggagggggatgggtagtggtggagggggccggctttgcaaaacttgggacccgggcctaaaggtgcctcctgctgctgctgctgctggtctttgccaccgccgccgccgcccccgtggtccttggtgcccacgccgccgccttgttcgtcttggggacttatatcagcgctgtgaagtctcttggggcagcggaaacgcagatgcgccacataggggaactcaaactggaaacgttggctgcattccaggcatgtgtaaggggacgaccctgcattcattttgttgtgggatctagaggggcagagcaagagtaactcagtcagttctttcccgtaccaaactagtaactcctcgtctttggcaatcctgcggagagagcggtagaacagctgtccgttttttatgtaggcttcaaggttctgctcttccttatctctggccgattggaccaaccgcagccacatgagaccttctgaggaaccatttgctgctgaggtgtctacccgaaagatatacggtactgttctcttgtcagtagacttgagagctatgaaagctatgctgtcatatagggaagtatggctcaggacacagggaccaaatatagcattctcagggatgtcgcaggtggtgtaaacgctggtaaaaatatctgtcagacattgttggacagccttggcatctccatcccagatgcctcgctggatgccagtatcctccatcacaggaataaggtcagtatagaatctcccaaataaggccacctggaaccgggaagatgcaatcgagtgtttccttttgcctattgtatcagtgtatttccatgtcaagaggtgttggtgttgccgccttttaggctcttccaagatgggctccggaaagcttttcacatccagcgggtggtggaggaggggatggagttgccgaggccgtctcgggagcctcgtttgtgcgctaagccacttagaggcgctgacttgcccctttagtgcagcagctgatgctaatgacttgaggtctttaacagcctgcaagttgactccttcaacggggctgcaacaccacgtcgctggggaatctcgggcttctttttcacagttcaattctctactcattatgaagtggaggcaagaataggcaaggattgtaacatatttgttctcttgaacttgctgagcgaaaagatgcttcccaggctgatttgatagtatctggggactgtggggctccttccccgggagcgcagctactgcgggcccctcggcggccgctctcccaccccaatcggagcctgccgaggagcccgtccgcctcgcgaaatggccccggtctctgctgcagcagctgggagggagggagcgaccgccggctgctgccgggcggcgtctgggggccgcgagccgagcgcaaggagaagccatctggagcctcggcagcgggcgggggtgggggtacaagagaaggggccaggctgctcggccccaggcgggcgcggggcagggctctggcgtgggagtggcgcccagtcgccccaagtactgcgtgtgtgtcgcgggaggggtggtgtggggaggtgtgtgagggtcatggcccctggggaggaggagcggaggcctgccgttctcaagtcccgccgattacagggcagcccggtacccgcaggtttagcaaaagagaggggatcctcctggcaaccaccagcccccctccagccattctccctccggggatggagagctgggcgaggacaacccaagcactcctacacgctcacacacccgctgtccgtcagaagtggtttgctcattttcctctcttcccaccttgtccatcccactccaggaaacat

SEQ ID NO: 18638 - RNA, 3044 nt, Homo sapiens
  source 1..3044: mol_type = other RNA
tgagtgtgtgtgtgtgagtgtgtctgtgtgtgtgtgtgggggggggtgtgtgtcccgggtaaatatttgaatgaggttcctgggaggagaggacgtgtgtgtgcgcgttgggggggcgggggggcggtgaatgtatgtgtctttgtgcagggtttcggggtgcaaggaagcggtggatgttctcgcgtgtttattcctgcaggtggcttaactgtgcttgcgcgcgcgtggaaagctggggtcctttccgagtcaattatgcgaggtcatgtgcctggagaggtggtggcgctccctgaaggactcattgcagatggggcacttgagtttctcctctcgccgccgcttcaccaagggctccatcgcatactcctttttgtggtgcgacctcatatggtacaccaggtcggaggtcatgcggaaggaggcattgcacttggcgcaccagttctgcgcgggcagacacagcgaggtgaaggagggcggcagcagcgtgagcgccgagggcagctgcagctgcaagggccccgcggccgccgccgcagccgcggctgcagcggcagcggagctcttgggccagaaggcggtggcgtacaggaaggggctctgcttaggcaggccgccgccgccgctcggcagggacccgcaacctccgttcaggtccgcggccccctggagcttcaccgctagagggtccgcggcggcgggatagagtctggtggggcccacgccgtcggcggggtggcatggctcgagcgcgcccagcttctggcccagcaccagcggggacagctgcgagaaagagcgtgctggctgcgagaaggcgcttttgcgctcgtccgacgcggcgccctggcccccgcccgcgccgcctgcggccccggcgcccgttccgcccccaccgctggtgctgcccgcgctgcccagctgcggcaccgaagtgaaggcgctgcccctcgcaggactgccgccctcgagccggctgggcagcgggcccccaggccgcggggccagcagcttctcggcgcccaccggtgacgcggccgcgggcgtggaggagccgccgccgccgccagcgtcctggtcctcggaggcgactcccgcgccgtcggctgtcccctcctcctgcaggctggccgcgcgggcagccttcttcacctccacgaaggcgctgcgcttcgcctcgcccgtctcgggacttggcggcgcgaagaggcggccgttctcttccaggccgaagtagctgcccgaggctcggtactgctgcggtgtgcacaccagatcctccttggaggccgggaggggccgctctacgaagcggccccggccccctaccagaccagcgccaccgccgccctccgccgcctcctccgggaatttcctctttcctttgccgccgcccgtggcgatgccgtcgggactcagctccgcctcctggtggccgccgccgccgccgctgccgctaccgctgctgaggctctgggctggggagcagctgctgcctccccgggagttttccagctccctggccaggttgtggaagtctgtggatggcttcgcgctgctgccgccggcggcagcggatgggttgctgctttccggggagggggatgggtagtggtggagggggccggctttgcaaaacttgggacccgggcctaaaggtgcctcctgctgctgctgctgctggtctttgccaccgccgccgccgcccccgtggtccttggtgcccacgccgccgccttgttcgtcttggggacttatatcagcgctgtgaagtctcttggggcagcggaaacgcagatgcgccacataggggaactcaaactggaaacgttggctgcattccaggcatgtgtaaggggacgaccctgcattcattttgttgtgggatctagaggggcagagcaagagtaactcagtcagttctttcccgtaccaaactagtaactcctcgtctttggcaatcctgcggagagagcggtagaacagctgtccgttttttatgtaggcttcaaggttctgctcttccttatctctggccgattggaccaaccgcagccacatgagaccttctgaggaaccatttgctgctgaggtgtctacccgaaagatatacggtactgttctcttgtcagtagacttgagagctatgaaagctatgctgtcatatagggaagtatggctcaggacacagggaccaaatatagcattctcagggatgtcgcaggtggtgtaaacgctggtaaaaatatctgtcagacattgttggacagccttggcatctccatcccagatgcctcgctggatgccagtatcctccatcacaggaataaggtcagtatagaatctcccaaataaggccacctggaaccgggaagatgcaatcgagtgtttccttttgcctattgtatcagtgtatttccatgtcaagaggtgttggtgttgccgccttttaggctcttccaagatgggctccggaaagcttttcacatccagcgggtggtggaggaggggatggagttgccgaggccgtctcgggagcctcgtttgtgcgctaagccacttagaggcgctgacttgcccctttagtgcagcagctgatgctaatgacttgaggtctttaacagcctgcaagttgactccttcaacggggctgcaacaccacgtcgctggggaatctcgggcttctttttcacagttcaattctctactccatgttagtttgatcctctcccagctttgagacccttctctggaactcagtggggtattgaggctttgacagcctggtgactgcagtcccaggaggccaggggaggattttgcttgttccactttagcaaggctctttggagtcctggcaaaaatacacatgtaggaaactgtagtgttattttggaagagtgggctggagagaggttgataaatgacaccccaggtggcttttatgacattatgaagtggaggcaagaataggcaaggattgtaacatatttgttctcttgaacttgctgagcgaaaagatgcttcccaggctgatt

SEQ ID NO: 18639 - RNA, 3161 nt, Homo sapiens
  source 1..3161: mol_type = other RNA
tgagtgtgtgtgtgtgagtgtgtctgtgtgtgtgtgtgggggggggtgtgtgtcccgggtaaatatttgaatgaggttcctgggaggagaggacgtgtgtgtgcgcgttgggggggcgggggggcggtgaatgtatgtgtctttgtgcagggtttcggggtgcaaggaagcggtggatgttctcgcgtgtttattcctgcaggtggcttaactgtgcttgcgcgcgcgtggaaagctggggtcctttccgagtcaattatgcgaggtcatgtgcctggagaggtggtggcgctccctgaaggactcattgcagatggggcacttgagtttctcctctcgccgccgcttcaccaagggctccatcgcatactcctttttgtggtgcgacctcatatggtacaccaggtcggaggtcatgcggaaggaggcattgcacttggcgcaccagttctgcgcgggcagacacagcgaggtgaaggagggcggcagcagcgtgagcgccgagggcagctgcagctgcaagggccccgcggccgccgccgcagccgcggctgcagcggcagcggagctcttgggccagaaggcggtggcgtacaggaaggggctctgcttaggcaggccgccgccgccgctcggcagggacccgcaacctccgttcaggtccgcggccccctggagcttcaccgctagagggtccgcggcggcgggatagagtctggtggggcccacgccgtcggcggggtggcatggctcgagcgcgcccagcttctggcccagcaccagcggggacagctgcgagaaagagcgtgctggctgcgagaaggcgcttttgcgctcgtccgacgcggcgccctggcccccgcccgcgccgcctgcggccccggcgcccgttccgcccccaccgctggtgctgcccgcgctgcccagctgcggcaccgaagtgaaggcgctgcccctcgcaggactgccgccctcgagccggctgggcagcgggcccccaggccgcggggccagcagcttctcggcgcccaccggtgacgcggccgcgggcgtggaggagccgccgccgccgccagcgtcctggtcctcggaggcgactcccgcgccgtcggctgtcccctcctcctgcaggctggccgcgcgggcagccttcttcacctccacgaaggcgctgcgcttcgcctcgcccgtctcgggacttggcggcgcgaagaggcggccgttctcttccaggccgaagtagctgcccgaggctcggtactgctgcggtgtgcacaccagatcctccttggaggccgggaggggccgctctacgaagcggccccggccccctaccagaccagcgccaccgccgccctccgccgcctcctccgggaatttcctctttcctttgccgccgcccgtggcgatgccgtcgggactcagctccgcctcctggtggccgccgccgccgccgctgccgctaccgctgctgaggctctgggctggggagcagctgctgcctccccgggagttttccagctccctggccaggttgtggaagtctgtggatggcttcgcgctgctgccgccggcggcagcggatgggttgctgctttccggggagggggatgggtagtggtggagggggccggctttgcaaaacttgggacccgggcctaaaggtgcctcctgctgctgctgctgctggtctttgccaccgccgccgccgcccccgtggtccttggtgcccacgccgccgccttgttcgtcttggggacttatatcagcgctgtgaagtctcttggggcagcggaaacgcagatgcgccacataggggaactcaaactggaaacgttggctgcattccaggcatgtgtaaggggacgaccctgcattcattttgttgtgggatctagaggggcagagcaagagtaactcagtcagttctttcccgtaccaaactagtaactcctcgtctttggcaatcctgcggagagagcggtagaacagctgtccgttttttatgtaggcttcaaggttctgctcttccttatctctggccgattggaccaaccgcagccacatgagaccttctgaggaaccatttgctgctgaggtgtctacccgaaagatatacggtactgttctcttgtcagtagacttgagagctatgaaagctatgctgtcatatagggaagtatggctcaggacacagggaccaaatatagcattctcagggatgtcgcaggtggtgtaaacgctggtaaaaatatctgtcagacattgttggacagccttggcatctccatcccagatgcctcgctggatgccagtatcctccatcacaggaataaggtcagtatagaatctcccaaataaggccacctggaaccgggaagatgcaatcgagtgtttccttttgcctattgtatcagtgtatttccatgtcaagaggtgttggtgttgccgccttttaggctcttccaagatgggctccggaaagcttttcacatccagcgggtggtggaggaggggatggagttgccgaggccgtctcgggagcctcgtttgtgcgctaagccacttagaggcgctgacttgcccctttagtgcagcagctgatgctaatgacttgaggtctttaacagcctgcaagttgactccttcaacggggctgcaacaccacgtcgctggggaatctcgggcttctttttcacagttcaattctctactccatgttagtttgatcctctcccagctttgagacccttctctggaactcagtggggtattgaggctttgacagcctggtgactgcagtcccaggaggccaggggaggattttgcttgttccactttagcaaggctctttggagtcctggcaaaaatacacatgtaggaaactgtagtgttattttggaagagtgggctggagagaggttgataaatgacaccccaggtggcttttatgaccgctttccagcggaagggggcatctttgcggcagaggcagcgttccccggggcgggggcgggacgccggggcagagccagccctgtagccccggccccggggtgctggcgccctcttctggctgctgtgcggccgctccctgcttctcgcgggtgctctggtccagaaactgttccgccctccgcgcccaggatgaaggggcagag

SEQ ID NO: 18640 - RNA, 3593 nt, Homo sapiens
  source 1..3593: mol_type = other RNA
tgagtgtgtgtgtgtgagtgtgtctgtgtgtgtgtgtgggggggggtgtgtgtcccgggtaaatatttgaatgaggttcctgggaggagaggacgtgtgtgtgcgcgttgggggggcgggggggcggtgaatgtatgtgtctttgtgcagggtttcggggtgcaaggaagcggtggatgttctcgcgtgtttattcctgcaggtggcttaactgtgcttgcgcgcgcgtggaaagctggggtcctttccgagtcaattatgcgaggtcatgtgcctggagaggtggtggcgctccctgaaggactcattgcagatggggcacttgagtttctcctctcgccgccgcttcaccaagggctccatcgcatactcctttttgtggtgcgacctcatatggtacaccaggtcggaggtcatgcggaaggaggcattgcacttggcgcaccagttctgcgcgggcagacacagcgaggtgaaggagggcggcagcagcgtgagcgccgagggcagctgcagctgcaagggccccgcggccgccgccgcagccgcggctgcagcggcagcggagctcttgggccagaaggcggtggcgtacaggaaggggctctgcttaggcaggccgccgccgccgctcggcagggacccgcaacctccgttcaggtccgcggccccctggagcttcaccgctagagggtccgcggcggcgggatagagtctggtggggcccacgccgtcggcggggtggcatggctcgagcgcgcccagcttctggcccagcaccagcggggacagctgcgagaaagagcgtgctggctgcgagaaggcgcttttgcgctcgtccgacgcggcgccctggcccccgcccgcgccgcctgcggccccggcgcccgttccgcccccaccgctggtgctgcccgcgctgcccagctgcggcaccgaagtgaaggcgctgcccctcgcaggactgccgccctcgagccggctgggcagcgggcccccaggccgcggggccagcagcttctcggcgcccaccggtgacgcggccgcgggcgtggaggagccgccgccgccgccagcgtcctggtcctcggaggcgactcccgcgccgtcggctgtcccctcctcctgcaggctggccgcgcgggcagccttcttcacctccacgaaggcgctgcgcttcgcctcgcccgtctcgggacttggcggcgcgaagaggcggccgttctcttccaggccgaagtagctgcccgaggctcggtactgctgcggtgtgcacaccagatcctccttggaggccgggaggggccgctctacgaagcggccccggccccctaccagaccagcgccaccgccgccctccgccgcctcctccgggaatttcctctttcctttgccgccgcccgtggcgatgccgtcgggactcagctccgcctcctggtggccgccgccgccgccgctgccgctaccgctgctgaggctctgggctggggagcagctgctgcctccccgggagttttccagctccctggccaggttgtggaagtctgtggatggcttcgcgctgctgccgccggcggcagcggatgggttgctgctttccggggagggggatgggtagtggtggagggggccggctttgcaaaacttgggacccgggcctaaaggtgcctcctgctgctgctgctgctggtctttgccaccgccgccgccgcccccgtggtccttggtgcccacgccgccgccttgttcgtcttggggacttatatcagcgctgtgaagtctcttggggcagcggaaacgcagatgcgccacataggggaactcaaactggaaacgttggctgcattccaggcatgtgtaaggggacgaccctgcattcattttgttgtgggatctagaggggcagagcaagagtaactcagtcagttctttcccgtaccaaactagtaactcctcgtctttggcaatcctgcggagagagcggtagaacagctgtccgttttttatgtaggcttcaaggttctgctcttccttatctctggccgattggaccaaccgcagccacatgagaccttctgaggaaccatttgctgctgaggtgtctacccgaaagatatacggtactgttctcttgtcagtagacttgagagctatgaaagctatgctgtcatatagggaagtatggctcaggacacagggaccaaatatagcattctcagggatgtcgcaggtggtgtaaacgctggtaaaaatatctgtcagacattgttggacagccttggcatctccatcccagatgcctcgctggatgccagtatcctccatcacaggaataaggtcagtatagaatctcccaaataaggccacctggaaccgggaagatgcaatcgagtgtttccttttgcctattgtatcagtgtatttccatgtcaagaggtgttggtgttgccgccttttaggctcttccaagatgggctccggaaagcttttcacatccagcgggtggtggaggaggggatggagttgccgaggccgtctcgggagcctcgtttgtgcgctaagccacttagaggcgctgacttgcccctttagtgcagcagctgatgctaatgacttgaggtctttaacagcctgcaagttgactccttcaacggggctgcaacaccacgtcgctggggaatctcgggcttctttttcacagttcaattctctactccatgttagtttgatcctctcccagctttgagacccttctctggaactcagtggggtattgaggctttgacagcctggtgactgcagtcccaggaggccaggggaggattttgcttgttccactttagcaaggctctttggagtcctggcaaaaatacacatgtaggaaactgtagtgttattttggaagagtgggctggagagaggttgataaatgacaccccaggtggcttttatgacctggggactgtggggctccttccccgggagcgcagctactgcgggcccctcggcggccgctctcccaccccaatcggagcctgccgaggagcccgtccgcctcgcgaaatggccccggtctctgctgcagcagctgggagggagggagcgaccgccggctgctgccgggcggcgtctgggggccgcgagccgagcgcaaggagaagccatctggagcctcggcagcgggcgggggtgggggtacaagagaaggggccaggctgctcggccccaggcgggcgcggggcagggctctggcgtgggagtggcgcccagtcgccccaagtactgcgtgtgtgtcgcgggaggggtggtgtggggaggtgtgtgagggtcatggcccctggggaggaggagcggaggcctgccgttctcaagtcccgccgattacagggcagcccggtacccgcaggtttagcaaaagagaggggatcctcctggcaaccaccagcccccctccagccattctccctccggggatggagagctgggcgaggacaacccaagcactcctacacgctcacacacccgctgtccgtcagaagtggtttgctcattttcctctcttcccaccttgtccatcccactccaggaaacat

SEQ ID NO: 18641 - RNA, 2992 nt, Homo sapiens
  source 1..2992: mol_type = other RNA
tgagtgtgtgtgtgtgagtgtgtctgtgtgtgtgtgtgggggggggtgtgtgtcccgggtaaatatttgaatgaggttcctgggaggagaggacgtgtgtgtgcgcgttgggggggcgggggggcggtgaatgtatgtgtctttgtgcagggtttcggggtgcaaggaagcggtggatgttctcgcgtgtttattcctgcaggtggcttaactgtgcttgcgcgcgcgtggaaagctggggtcctttccgagtcaattatgcgaggtcatgtgcctggagaggtggtggcgctccctgaaggactcattgcagatggggcacttgagtttctcctctcgccgccgcttcaccaagggctccatcgcatactcctttttgtggtgcgacctcatatggtacaccaggtcggaggtcatgcggaaggaggcattgcacttggcgcaccagttctgcgcgggcagacacagcgaggtgaaggagggcggcagcagcgtgagcgccgagggcagctgcagctgcaagggccccgcggccgccgccgcagccgcggctgcagcggcagcggagctcttgggccagaaggcggtggcgtacaggaaggggctctgcttaggcaggccgccgccgccgctcggcagggacccgcaacctccgttcaggtccgcggccccctggagcttcaccgctagagggtccgcggcggcgggatagagtctggtggggcccacgccgtcggcggggtggcatggctcgagcgcgcccagcttctggcccagcaccagcggggacagctgcgagaaagagcgtgctggctgcgagaaggcgcttttgcgctcgtccgacgcggcgccctggcccccgcccgcgccgcctgcggccccggcgcccgttccgcccccaccgctggtgctgcccgcgctgcccagctgcggcaccgaagtgaaggcgctgcccctcgcaggactgccgccctcgagccggctgggcagcgggcccccaggccgcggggccagcagcttctcggcgcccaccggtgacgcggccgcgggcgtggaggagccgccgccgccgccagcgtcctggtcctcggaggcgactcccgcgccgtcggctgtcccctcctcctgcaggctggccgcgcgggcagccttcttcacctccacgaaggcgctgcgcttcgcctcgcccgtctcgggacttggcggcgcgaagaggcggccgttctcttccaggccgaagtagctgcccgaggctcggtactgctgcggtgtgcacaccagatcctccttggaggccgggaggggccgctctacgaagcggccccggccccctaccagaccagcgccaccgccgccctccgccgcctcctccgggaatttcctctttcctttgccgccgcccgtggcgatgccgtcgggactcagctccgcctcctggtggccgccgccgccgccgctgccgctaccgctgctgaggctctgggctggggagcagctgctgcctccccgggagttttccagctccctggccaggttgtggaagtctgtggatggcttcgcgctgctgccgccggcggcagcggatgggttgctgctttccggggagggggatgggtagtggtggagggggccggctttgcaaaacttgggacccgggcctaaaggtgcctcctgctgctgctgctgctggtctttgccaccgccgccgccgcccccgtggtccttggtgcccacgccgccgccttgttcgtcttggggacttatatcagcgctgtgaagtctcttggggcagcggaaacgcagatgcgccacataggggaactcaaactggaaacgttggctgcattccaggcatgtgtaaggggacgaccctgcattcattttgttgtgggatctagaggggcagagcaagagtaactcagtcagttctttcccgtaccaaactagtaactcctcgtctttggcaatcctgcggagagagcggtagaacagctgtccgttttttatgtaggcttcaaggttctgctcttccttatctctggccgattggaccaaccgcagccacatgagaccttctgaggaaccatttgctgctgaggtgtctacccgaaagatatacggtactgttctcttgtcagtagacttgagagctatgaaagctatgctgtcatatagggaagtatggctcaggacacagggaccaaatatagcattctcagggatgtcgcaggtggtgtaaacgctggtaaaaatatctgtcagacattgttggacagccttggcatctccatcccagatgcctcgctggatgccagtatcctccatcacaggaataaggtcagtatagaatctcccaaataaggccacctggaaccgggaagatgcaatcgagtgtttccttttgcctattgtatcagtgtatttccatgtcaagaggtgttggtgttgccgccttttaggctcttccaagatgggctccggaaagcttttcacatccagcgggtggtggaggaggggatggagttgccgaggccgtctcgggagcctcgtttgtgcgctaagccacttagaggcgctgacttgcccctttagtgcagcagctgatgctaatgacttgaggtctttaacagcctgcaagttgactccttcaacggggctgcaacaccacgtcgctggggaatctcgggcttctttttcacagttcaattctctactccgctttccagcggaagggggcatctttgcggcagaggcagcgttccccggggcgggggcgggacgccggggcagagccagccctgtagccccggccccggggtgctggcgccctcttctggctgctgtgcggccgctccctgcttctcgcgggtgctctggtccagaaactgttccgccctccgcgcccaggatgaaggggcagaggggaggaaggtcaagaaagagagagggttgggtaccggaacgctcaggctcctccttccccgcccttcgc

SEQ ID NO: 18642 - RNA, 780 nt, Homo sapiens
  source 1..780: mol_type = other RNA
tgagtgtgtgtgtgtgagtgtgtgaaagtgtgtgtttcaaaggagacttctgggatgatggcgtaaatgtgtatgtgagtgtgtatgtgtttcaagggagatttctgggatggtgtcatgaatgtgtgcgtgtgtgtgtgtgtgtgtgtgagggttcgtgagtgtgtgtgtttcaaggaagatttctgggatggtgttgggaatgtgtgtgagtgtgtgtgtgtgtgagtgtgtatgtgtttcaagggagatttctgggatgatggtggtgtgaatgtgtatgtgtgtgagtgtgtgtgtttcaagggagatttctgagctgacagtggtgtcaatgtgtgagtgtgtgtgcatgtgagtgtgtgtgagtgtgagtgagtgagagcatgtgtgtgtgtgagagtgtgtgtgagagtgtgtgtttcaagggagattcctgggctcgggctcttggacattgggcagaaggctgtgtcctctcctttgaccagtctctgttgtgtttcttccctgagctcatcaagagcagcctcagccatcccaagagcccccagagctgtttgtgggcagctgagcctgtgcagcccagcctcacccttgtcacagtgggccctaccaccatgtttggcccccatgagccatggcattttcacagtcaccctgcatagaaccaaggctggtcaccctttcacagatggagacacaaggaggatgtagcagtagggtgagatcagatcacgaggcggcttttgcttgttttttgataagaaagttttattt

SEQ ID NO: 18643 - RNA, 32 nt, Homo sapiens
  source 1..32: mol_type = other RNA
tgagtgtgtgtgtgtgagtgtgtgagtgcgcg

SEQ ID NO: 18644 - RNA, 33 nt, Homo sapiens
  source 1..33: mol_type = other RNA
tgagtgtgtgtgtgtgagtgtgtgagtgcgcgc

SEQ ID NO: 18645 - RNA, 114 nt, Homo sapiens
  source 1..114: mol_type = other RNA
tgagtgtgtgtgtgtgagtgtgtgagtgtgtgtgtgagagagagaaagacagagagagagagacaaaagcaccagtttgagtctctcaagtcctcggttagctttcatgtctgt

SEQ ID NO: 18646 - RNA, 4309 nt, Homo sapiens
  source 1..4309: mol_type = other RNA
tgagtgtgtgtgtgtgagtgtgtgcatgcacatgcccactcccacagccttctcatacatccaggcagcccgctggcaccccagcttcagctcagccagccttcctccccgtaaacctggagcagctaaaattagtatgaaaatggtagtgttcggttaaaaggaaggggggtgggaagagatgagggtacccatgagtgctattttatttctcagtgagaggataaagtgatttttcctacataatttttgatgtagaggctaaattaggccggagaagagggacaaagcaactttcgccctcattagtattctggccgcgttggcccaggcacggcagttatgtatttttgcaagtatgcatataatttattgtggagaacacaatttacatggtagtcgatgcctgttttatagcctcacaaatagatgtatgaactcaagcatataatggcccaaccagcaggcgcaaatacgttctaaatcttctaaatgtgcttcacaaaaatgtaactgaggaatataaaacagatcaattcttgcatgttatatattggtttttgatttacaaatctaatctgggacatttcttcagaaatgaggggatttttcccccacgctttcccctcctcttcttccacaacttctctgtgcacagacctcgcctgctggtcaggtgccagcaggcattgccacttctgggatatgcctaggtgcccgtgtgtgtgctcatgtgtgggggccacgctcttgcctgtctgcctgggtgtgcactcgtatgtgtgtcaggaatctgcagacctcgggtggaagggagagagtggtttctctccatctgtgtgacctcccccatttgaggctgaaaatttggggagaagggctgatgagaggaccccatgagggtgtgggcatctctcagatgtgttccctctgggcttctgcttaaacggcctattttcttctgagacccaagctgtcttcatgacttattggagcagaaaagggaatgaggatcctagggatgaaattaaactaatatgtgttgagttgcattttaaatgtgcattttatcagaaatattttaatcaacctatctttaggtacatggctttttaaaaagcccattccatcaatagttgaacagacacataaatgatggtgtactcataaaatggaatatgatacagctaagaaaatttgagccaacgattgcttcctacaacagcatggggaatctcacaaacagaatgtaaaatgcaagaagccggacccaaaagaggacctgctacttgattggatttatcaagcacgaactgaacccaactattgtgtgtagagatggcaaaactatcaaggagagcaagagtatttgccataaaggtcagaatggtggttttctttggggaggaggattggctagagtacaggaggggcttctggggaggtggtaatgttcctcttgaccaagtggtggtttcatggatattcacttggtgataaattactgagcggtactttttaaaaatccacttttctgtatgtgtcttatattttgcaatcaaagcatttacaaaaatagcccttaaggacttataataaaaagcaggcaccccagctccacccaccccagccctgtttccctgaaggcaactactggtaaccatttccggatgttctctccaatctctagaaatgttgtggagtttctttcgaatctatcagtgaaattgtataatcctttttatttctgtaaggtcagtggcaaggtctccacttccattcctgactttagtaatttcagttttctctctctttttttttttctcggtcagtttagctaaaggtttgtcaattctgtagatcatttcagacaaccaacttttggttttgctgatttttctctatcgtttttctgttctctgtttcatttatctctgctctaatttttttatttgcttgctttggatttagtttgctttttttttttttagtaaggtggaaggttattgatttgagatcttctattttaaggtaggtgtttacagctataaatttccctctgagcactgcttttactgcatcctgtaagttttagtatgttgtgtttttgttttcattcgtctcaaagtattttctaatttcccttatgatttattttttgaccctttggttaggagtgtgtcgtttaatttttacatatttgtgaattttcaaatttccttctgtttttgaccttctaatttcattactctgttgtcagagaacatattttgtgtaatttcaatttttctaaatttattgagatttgatttgtggcctaagatatgatctatgctagagaatggtccgtgtgcacttgagaagaatgtgtattctgctgttgctgggtggaatgtgctcttcaatcgccgttagaaagcagtgtctgttaggtctagctggtttacagtgtttttaaagtcttctatttccttactgatctcctatctagtgttccatccattacatcgatgaaattttttctcatctatgtgatacttataaggtacaagtcacagccctaatttcaggaggttcacaatccagtgggggtgggggagcttcacttctacctagctgggccaccccatccctgatctccaatatgggaggatcgccctcatccccatactgtcttgcagcctggggtcttgggctgtgcaactccccatcagcctcaagtatctccatctctcccattcccacggttactaaccctggtgcaaacaaagcagaactggaagaggtctcgaagaccacgtggaggtcaatgcccttgtggtacagatagggaaactgaggcccagagaggggcaagatctttttctaggtctcctggagagccaggcccagtgatgtcctatcaatcatctgctcagcccacagcaccatgatctagtggctatcgagaaaaagggacctgttgatgtcaccctctgtgtcatttccatttgtagtatggggtggtggcagacaaggccagtattagagggggtgagggggctgtgttgaacacacatcccagagcacttagaagacctacgcttccatcctagcttaaccactctgagctgtgtgagcttgagcaagtcactctcctgctctgaacttcagtttccttatatgcaaaatagaaaacatcgtaagcactgccaccattcattgagtccctaccaagtacccagtactgtactcatacaatttcattcagtcctcctgaccgccttgggagaggtcagtacctttggcataggaagaaagagaggccccataaagcaaaccacccacccaaagccacaggtattcaaccctcaccctcttaaggctccaaagctaaagcacagaagccgcccggccacatggccctccatccacccttgcagtgtgggtttacatatttacgggaggaggcggggcgcagttaaagagggactgagtgtcagctgacgctcaccatgggattactgttaatttcctcaggtgtgatcctggcatggccagttagtgagaggtacttactgaagtcattccacatgaagtcacctgatatctgggatttgttttcaactacctgtgtgcctgctgataagcactggtcagagccaatcctcgctcttcacgaagtgccctccgtgggtggtctctctggtgccacttgctctgttgctctgttctgctcatttggtcagcttccctctttaagtgaggggctcagagcagacccagggctctgggtgaggccccctcatgctgagccattctcttcctcaagggatctgaacgtcttggttctgctcctgcaacctgggagtaaggtagctttagagcagccttctcttgctacccagatgaggtaagaagagcatgatccaggctgctggaagctgcaagtcagaagacacaagcgttcagtcctggtgtctctgtgcggtggtgtggtcttgggcggtcctttaactctcctaggcctcagtttcctcataggttgaaaaatgcagctccagagagaaaccagtgggaggccaaggaattcaagttgagccagggtccaggttccagctaagaagggagtgacctgtgagtggatgaagaggcggctccccggggccttcgctggaagaggtggggaaaaggatgtcagattacagagcaggaggcttcacgctccggtgccggcacctaaatcactgtctccgcggccgcgctcaaggttgctcccgagccggccgccgccgagcagccgcgggaactccggccgagcccccacccc

SEQ ID NO: 18647 - RNA, 4013 nt, Homo sapiens
  source 1..4013: mol_type = other RNA
tgagtgtgtgtgtgtgagtgtgtgcatgcacatgcccactcccacagccttctcatacatccaggcagcccgctggcaccccagcttcagctcagccaggcttcctccccgtaaacctggagcagctaaaattagtatgaaaatggtagtgttcggttaaaaggaacgggggtgggaagagatgagggtacccatgagtgctattttatttctcagtgagaggataaagtgatttttcctacataatttttgatgtagaggctaaattaggccggagaagagggacaaagcaactttcgccctcattagtattctggccgcgttggcccaggcacggcagttatgtatttttgcaagtatgcatataatttattgtggagaacacaatttacatggtagtcgatgcctgttttatagcctcacaaatagatgtatgaactcaagcatataatggcccaaccagcaggcgcaaatacgttctaaatcttctaaatgtgcttcacaaaaatgtaactgaggaatataaaacagatcaattcttgcatgttatatattggtttttgatttacaaatctaatctgggacatttcttcagaaatgaggggatttttcccccacgctttcccctcctcttcttccacaacttctctgtgcacagacctcgcctgctggtcaggtgccagcaggcattgccacttctgggatatgcctaggtgcccgtgtgtgtgctcatgtgtgggggccacgctcttgcctgtctgcctgggtgtgcactcgtatgtgtgtcaggaatctgcagacctcgggtggaagggagagagtggtttctctccatctgtgtgacctcccccatttgaggctgaaaatttggggagaagggctgatgagaggaccccatgggggtgtgggcatctctcagatgtgttccctctgggcttctgcttaaacggcctattttcttctgagacccaagctgtcttcatgacttattggagcagaaaagggaatgaggatcctagggatgaaattaaactaatatgtgttgagttgcattttaaatgtgcattttatcagaaatattttaatcaacctatctttaggtacatggctttttaaaaagcccattccatcaatagttgaacagacacataaatgatggtgtactcataaaatggaatatgatacagctaagaaaatttgagccaacgactgcttcctacaacagcatggggaatctcacaaacagaatgtaaaatgcaagaagccggacccaaaagaggacctgctacttgattggatttatcaagcacgaactgaacccaactattgtgtgtagagatggcaaaactatcaaggagagcaagagtatttgccataaaggtcagaatggtggttttctttggggaggaggattggctagagtacaggaggggcttctggggaggtggtaatgttcctcttgaccaagtggtggtttcatggatattcacttggtgataaattactgagcggtactttttaaaaatccactttctgtatgtgtcttatattttgcaatcaaagcatttacaaaaatagcccttaaggacttataataaaaagcaggcaccccagctccacccaccccagccctgtttccctgaaggcaactactggtaaccatttccggatgttctctccaatctctagaaatgttgtggagtttctttcgaatctatcagtgaaattgtataatcctttttatttctgtaaggtcagtggcaaggtctccacttccattcctgactttagtaatttcagttttctctctctttttttttttctcggtcagtttagctaaaggtttgtcaattctgtagatcatttcagacaaccaacttttggttttgctgatttttctctatcgtttttctgttctctgtttcatttatctctgttctaatttttttatttgcttgctttggatttagtttgctttttttttttttagtaaggtggaaggttattgatttgagatcttctattttaaggtaggtgtttacagctataaatttccctctgagcactgcttttactgcatcctgtaagttttagtatgttgtgtttttgttttcattcgtctcaaagtattttctaatttcccttatgatttattttttgaccctttggttaggagtgtgtcgtttaatttttacatatttgtgaattttcaaatttccttctgtttttgaccttctaatttcattactctgttgtcagagaacatattttgtgtaatttcaatttttctaaatttattgagatttgatttgtggcctaagatatgatctatgctagagaatggtccgtgtgcacttgagaagaatgtgtattctgctgttgctgggtggaatgtgctcttcaatcgccgttagaaagcagtgtctgttaggtctagctggtttacagtgtttttaaagtcttctatttccttactgatctcctatctagtgttccatccattacatcgatgaaattttttatctcatctatgtgatacttataaggtacaagtcacagccctaatttcaggaggttcacaatccagtgggggtgggggagcttcacttctacctagctgggccaccccatccctgatctccaatatgggaggatcgccctcatccccatactgtcttgcagcctggggtcttgggctgtgcaactccccatcagcctcaagtatctccatctctcccattcccacggttactaaccctggtgcaaacaaagcagaactggaagaggtctcgaagaccacgtggaggtcaatgcccttgtggtacagatagggaaactgaggcccagagaggggcaagatctttttctaggtctcctggagagccaggcccagtgatgtcctatcaatcatctgctcagcccacagcaccatgatctagtggctatcgagaaaaagggaccagttgatgtcaccctctgtgtcatttccatttgtagtatggggtggtggcagacaaggccagtattagagggggtgagggggctgtgttgaacacacatcccagagcacttagaagacctacgcttccatcctagcttaaccactctgagctgtgtgagcttgagcaagtcactctcctgctctgaacttcagtttccttatatgcaaaatagaaaacatcgtaagcactgccaccattcattgagtccctaccaagtacccagtactgtactcatacaatttcattcagtcctcctgaccgccttgggagaggtcagtacctttggcataggaagaaagagaggccccataaagcaaaccacccacccaaagccacaggtattcaaccctcaccctcttaaggctccaaagctaaagcacagaagccgcccggccacatggccctccatccacccttgcagtgtgggtttacatatttacgggaggaggcggggcgcagttaaagagggactgagtgtcagctgacgctcaccatgggattactgttaatttcctcaggtgtgatcctggcatggccagttagtgagaggtacttactgaagtcattccacatgaagtcacctgatatctgggatttgttttcaactacctgtgtgcctgctgataagcactggtcagagccaatcctcgctcttcacgaagtgccctccgtgggtggtctctctggtgccacttgctctgttgctctgttctgctcatttggtcagcttccctctttaagtgaggggctcagagcagacccagggctctgggtgaggccccctcatgctgagccattctcttcctcaagggatctgaacgtcttggttctgctcctgcaacctgggagtaaggtagctttagagcagccttctcttgctacccagatgaggtaagaagagcatgatccaggctgctggaagctgcaagtcagaagacacaagcgttcagtcctggtgtctctgtgcggtggtgtggtcttgggcagtcctttaactctcctaggcctcag

SEQ ID NO: 18648 - RNA, 4200 nt, Homo sapiens
  source 1..4200: mol_type = other RNA
tgagtgtgtgtgtgtgagtgtgtgcatgtgtgcatttctcatatggaacagacaaatgtaaaataactgaatacagaagaagtaacatgagatgaacaaacttgtgaaataattggataccttcaatagaaatctatgatcaacatggctcaaatacagagtgctctagggagtggaaggtaaggttagaaaggtcagtgagagcttagtgaagaacagccctgctggaatatgccaggccattgggtccagactttattttcagagagtgggaaatccttaaaacttttcaccaggtaagatgtatattgtatgtattaaattccccttcctccagaaagttttcttctaaaacttatctgaaggaaatagcttgaataagtgcacaagaaatttgatataagaatgtttctgatttttttttcttacgaaaatgtgagaggttgaaaacaattgcataggagggctttaaaatacagtatgctatatccattggatggactattatatagatcttgtgatgacatggaaagatatctgtaatatgtcattaaatagagaaagcagattacagaaaaatatgaagagtacaattttagcagtctaaccacatgtaattttagatgcattaaaaatatggaatgataacattcaaatcattcaacatcctcagaaattatatccttttcatatgtttctgtttggtttgaagtttttacaataagcaaaagcaatataggcatacccattttgaaaaagaattttatatcagaaacatcactgtagcatattgtagggattgatatggaagagtttgttagttggaacaaaaattgaaggcactgtaacaaagatacacaaattacagtgtttctgacagatacattgatttccctcttgtgtaacaactcgagtaacatccagctctgtgtccacaagtccaccagggacccaagctgacagggcaggtgtcctttccccaaaactggtgttcaagattttccggttcttgccatttccagaaaatgggaaggaaaagggagaaaagagttccggacaagattcttttgttgaaatgacttggaccctgtacacatcacttcctcttatgtcttattactgagttatagaattaactgagggttggaggaagggtcgacaatcagcaatctgccacaaggagcaaaaaaactctaaataggggagattgttttgcagcttgatgtaatcatcaagctaaaagatgagtttgtgcttttgttattattacttatctttaaatgagcttccggtgcatataattggattaactgtattccttgtttcaaaatatatgttgatcattggtttatacaagtttctcacttgcttttttgtttattataaaataaattgctgccctaaataaaaatgaaattggttgggttttgccacataataaatcattcaaaaatcagtggcttcaaacaacaatgatttactggttcatgattttgtgggctggcaattcacctgggctcacctgggtcattcctctggtctgggcaggtttggctggatagtctgagatagcctcattcacagttgtctggaagttgttgtggaccattggttaatagtcagctggggttacagaggtggtgggtccagatttttctaccaggctagctcaagtgtgttcacatgacaatgactgtagtgtttccattcattcatttgttccatcaagtcttcctatgccctggaggtacacagcaccagtggagcaggcaaacttggacacagataattatgatatcacattctaagaattttcacaaagataacaggatatgggagcacttggagggagcagttatccctggcaaagtggaggaatgtattaccgaggaagaaattttccagttggtcttaacaaatgaattagagatgctcccgtgcagaaggagagagagaatggatgcacgtggaagaaaggtgttgcagccagatacaaaggttggagaaaggatggggtcgtccatctggagccttcctccaccttgtatggaggcaggaaatgagcctggagaaagtagttgtaaaggcagcttgaactcaaccccatacacagaggaggccatcagattctaggcatgatcaggtgtctgaagtgctgctgaggatttctttggaaggacctactggaaacaggcattcctcttccctatttcatttttcttttatcctgaattgctgctccctgccagtcacatggtacctatcttggagagcagccagccagggcaaaatgcctaacttcatccctggtggctgcagcatcttcatcaaatccagaagcccaaaccattacatgttttagatacagcaaagcacaggggaagagtacaaaagctaagttgagtccttgccctagtgcttacaaacacaaaatttgtgtcctcagtctcaactatcccacttgaaatgttctcacttctgtgtttttgatcacactcccctacctacaacaagaattcccttcttcctgcatattcatcaggtccatataaaaagttttctaaaaagagtaaaggatgtgattgtccccttctttacactctcagaacactttaccctatggaagtcacttctgcctgaagatgtactcatgtgtaacagaagaggatagtcttgcctggaatgcaaactccacataccagggtcaccatctctacatttcctggacgtaggtaacacttggctttcaatagctgcataattactgtgaagtgacgtaagcacagacctaggatctagtcaggcctggtttcaaatcttgactgtaatacttcctaagcaccacttatcactaatcaggtcatttgacctctaattctcaagcagcattggcaggttagagatcatggaggtaaagctcccagccgattctcaggacatggtggggctccacaaatggtgtctgctaataaatgtccccttttttcccttgtcttctctttgccacttgcaacaagggaacttatattttcctgatatactggatgactgtgggatgaaaatctaaaaatcaaaaatctaaataaaatagatgacagaactcttgcagaccctttcatccccatgaaaaatgatcacaaggaactaaaatacataatcaaggggagagataaatgtcatgcaaaatttccatctcaaaataaaaggcgagctgcaccacattcttccccataatcacatcgtggaaacatgtgcaacactgcatcaagcctggagtatattatgaacccctgcagacacagaaattttgtgagctgtaggttgcagaaacccacagagctgggaaagcagaggtttaatggtattttaaatgttttgactatgcaggaggcagaatctgcagtctaatcattttcagaatacttgatgcactgtaggcaaccatgggacttgtgtactccccagcaatctgcacctagaatggggcaagttataagggaagagaagggaaggaaaggggatggcaagtatatggagcacctactatgtgtgtggtacgctccctcggctacttcccttaatcttcccagtatccctggaaggtaggttttctgagctacacctctggtcttaaaaggtagctgatatgagcttctgagagttatgagaaaaataattctaaatctcatttatgtgtgaaagttaaatcattccatacacccatgttcatagcagtggtattcaaaataaccaaagggtagaattaaccctactgtctatccgtggatgaatggataaacaaaacacagtacttacatgcaataggctgcttttcagccttaaaaaggaagaaaactctgacacatgctatgatatgaataaatcctgagggcactatactaagtgaagtaaactggtcataaacaatcaaatactgtatgactccacctatatgaggtatctagaatagtcaaattcatatctcctatcaagagtagagtggtggttgtctggggctaggggaggagagaatagggagttgtttaatggatagaaagtttcagttttgcaaaattaaagagttctggaaactggttgcacaacaacacgaatatacctaacattactaaatcatacacttaaaattggttaagaggctgggcacagtggctcacgcctgtaatcccagcactagagggt

SEQ ID NO: 18649 - RNA, 621 nt, Homo sapiens
  source 1..621: mol_type = other RNA
tgagtgtgtgtgtgtgagtgtgtgggtgtgggtgtttagagggcggggcagccaccgcccaaacatcacctcgggtcagatggttttctgggctcataacctaatgctcagtgcccccccctccttttattggccacttttatgattattatttttaccgacagctccaagcagaggcctgtgggcctgggcctcctggaaggcaatcactgttctgccattcagcctgggaggccaaaggggctgtctgcagcagcctgggccacccgagtctatatttggaagcaaattccacagccacttcctgggaactgggaaaaaggtgcattccaaacaaagaagatattggtgcagaccacatggatcctggggacaacatcctcttctcccaggagtatcagtctccattcatttatgtcaaagcctgatttccccttccacacccctggttgtgggtggatggatgaagaaggcctttacttggagcctaagccctggcgcgcgcgcaccacggcgcgaactgctccatcaagcatccactggcctccagccgcgtttccggttgtagcactgggcgcccccagagtggacccgataagctatcggcgcggcccaggaggg

SEQ ID NO: 18650 - RNA, 25 nt, Homo sapiens
  source 1..25: mol_type = other RNA
tgagtgtgtgtgtgtgagtgtgtgt

SEQ ID NO: 18651 - RNA, 129 nt, Homo sapiens
  source 1..129: mol_type = other RNA
tgagtgtgtgtgtgtgagtgtgtgtatgtgagtgtgtgtaattaaatgtgtgtacatgtggaattcaaatgaatgctgcattaatcatcgacacaaatttggggtacttcctgtgttaggcaccgttga

SEQ ID NO: 18652 - RNA, 294 nt, Homo sapiens
  source 1..294: mol_type = other RNA
tgagtgtgtgtgtgtgagtgtgtgtgaagagtgaggagggggagtgtggggttttttttttttgaacaaaaacaaaccgaaagggcgcctgggagtcgtagtcccaacggcctctctggcctcccccgctccggaagaatatggccgcgtgaagcgcgtggaccacacttcccggcgtgcccggcggcccccttccgctctccctctcgcgtcctccgcctagcaccgacctcagctaggaacggggacgggtcgctgttcggggaaggggctgggtggagtctcgcgaggtgc

SEQ ID NO: 18653 - RNA, 151 nt, Homo sapiens
  source 1..151: mol_type = other RNA
tgagtgtgtgtgtgtgagtgtgtgtgactctgtgtgtctgtgtgtatgtgtgtgtgtatgtctgcacccagctctggtctcccggaggcttcctgctttgtgtctcccccacctcctgcagccgtggccaacacacacacttcctgaaaac

SEQ ID NO: 18654 - RNA, 231 nt, Homo sapiens
  source 1..231: mol_type = other RNA
tgagtgtgtgtgtgtgagtgtgtgtgagtgttggccaagtcgtccctgcgcggcgacagcgcggcttgggctctccgcccggcggctcgcgggctccccctccgccgccgccgcccgcctagctcccgctctcggtcgcggtctgggctcctgcgcgtctcccccgcagccgccgagctcggcccgcgttcagcgaggagcgcagctctgcctcaccttgccgctgggagc

SEQ ID NO: 18655 - RNA, 244 nt, Homo sapiens
  source 1..244: mol_type = other RNA
tgagtgtgtgtgtgtgagtgtgtgtgagtgttggccaagtcgtccctgcgcggcgacagcgcggcttgggctctccgcccggcggctcgcgggctccccctccgccgccgccgcccgcctagctcccgctctcggtcgcggtctgggctcctgcgcgtctcccccgcagccgccgagctcggcccgcgttcagcgaggagcgcagctctgcctcaccttgccgctgggagcccaggctccgtct

SEQ ID NO: 18656 - RNA, 15291 nt, Homo sapiens
  source 1..15291: mol_type = other RNA
tgagtgtgtgtgtgtgagtgtgtgtgatggggaaaaaagaacaattgtgtgattcacaaatggcataaaacactgattgtattacaaataagaatggtggcactctagtaagtaagataatggaatgtcaaaggaaacaaactttagaatacaaacatggaaaacatgctaaaatattaatcaagctatagcttgtggcatgtgattcttctttcccaagtattttgagagtgtcatttacccccagtagaattctatatcaactgcctctaagtccttttcctattccttcttttttttttttttgagacggagtctcactctgccacccaggctggagtgcaatggtgggatctcggctcactgcaacctccgcctcctgggttccagactaccttgtctggaaaggccctgcttggtgttttctatttaaaggggaaaaccaaacatgttatgttgatagcaatgcctggctctattaaagataaatccttcatttaatttccttattgtaattcagactagcaggattctcctgcctcagcctcaggcgcctgccaccacgcctagctaattttgtatttttagtagagacagggtttcaccatattggccacgctggtctcaaactcctgaccttgtgatccacctgccttggcctcccaaagtgctgggattgcaggcatgagccactgctcccggcctattctttcttttttaaagagggaatggggttggaccctgggctaagaaatgagaaagctcctggaaaaccttaattgcaattaattactatagaagatcaagtctgttgctagcaaaaccaaagcttccttttgttaaactccctgggatcaaactgtatccatgaactgggtcggactgtctatgccaaaattctttcttcattacaaactaaccagtgtttttaccaaatcccacaccaaaaccattttctttacaggaaagactacattgtctggaaaggccctgcttggtgttttctatttaaaggggaaaaccaaagacactatgttgatagcaatgcctggccctatttaaggataaagacttcatttaatttctttactgtaattcagaagcaacttccaagacttctctaagttactgagaataggtgtgcctttgggtctgggacaacattatcatataaatttagattacagagacgctcgtcttaggtctcttctgtaggttcaaatagcaatagctgctcttttactctgcaaatattaaacaattgtaaggtttctgtccaaggatcccagcaaggaagccttatcctaaatcccccctcactatatattctcacaatcctactagtctatttctttacaaagacctccagtttctacagattctgacaataaagagtcacgtatgcaacatttttgcagtctttccttctttggttctaaaaagactattaaaggactaacttaagagatttttgtttgttttcccaaccaaaaatgaaataaagatgaaataaagccatgaaataaagatgaaagttttgtcttttatttttaaaattattattattttttgagacggagtttcactcttgtcgcccaggctggagtgcagtggcatgatctcggctcactgcaacctccgcctaccgggttcaaacgattctctcgcctcagcctcccgagtagctgggattacaggcgcccaccaccatgcctggctaatttttgtatttttagtagagacgggttttgccatgttgtccaggctggtctcgaactcctgacctcaggtaatcagcctgcctcggcctcccgaagtgctgggattacaggtgtgagccaccgtgcccggccaagatgaaagttttaggcactaaatatcagagtaatctccctctctagtctctggtgttgcctcttcaacatcaaacataaaattatagatagcataccgccaatttttggaaagaataaaatttaaaaagcaaggctctaatgaccaacacttccatctgttttctacgcataacgctgttcatggcaattcttttttgggatgatctattactgcacaacgatttttttttttttttgagacagagtctcactctgttgcccaggctggagtgcagtggcacgatcttggctcactgcatcctccgccaccacacccggctaatttttgtatttttagaagagacagggttttgccatgttggccaggctggtcttgaactcctgacctcaggtgatctgctcacctcagctgcccaaagtgttgggattacaggtgtgagccactgcacctggccacaaagctttctttctaaagaggtgaactaaacatgaacaagccatcaagtacttcactgcggtcaagctgtactgatgtcaggtagcaggatttgtggagccaaccagttaaaacagcaaaataagctctatatgccaggtttctatgaactttcagaaggaaaaagaaaacacaggaccagaggcacctttttttgtttgtatgtttgttttgagatggagtcttgctctgttgccaggctggagtgcagcggtgcaatcttggctcactgcaacctccgcctcccaggttcaagtgattctcctgcctcagcctcccaagtagctgggactacaggcgtgtgccaccacacccagctaatttttgtatttttagtagagatggggtttcagcatgttggccaggatggtctccatctcttgacctcgtgatccgcccacctcggcctcccaaagtgcagggattacaggcgtgagccaccatgcccagcccagaggcaacttttaaaatgttggttttcaggaactacatgtctgctaaccttggacatgttgaaatgtaatgaatacaactattaaggttataagcgcaataaatatccttaaaaggggacatacaatcacagcaaaaatattttgctttttttttttttgagacggagtcttgctctgtcgcccaggctggagtgcagtggtgtgatcttggctcactgcaacctccgcctcctgggttcaagccattctcctgcctcggccttcccagtagctgggattacaggcacgtaccgccaagcccagctaatttttgtaattttagtagagacagggtttcaccatattgggcaggctggtctccaactcctgacctcgtgatccgcccgcctcagccgcccacccaaagtgctgggattacaggtgtgagctaccacgcccagccacattaatttgcttttaattagtagtaacaaattcttataatcagagtacaaatctgtactatctgtatacaattagtacttgatgtgtgcggggctgaagtatctcagaatagtatatcatagggcaaactaatgtaactggcaaaaatgcaaaaagaaatgaaatggctaatctctacaagaaatcacatgctgatctattttaaactgtaaaactttacatcatataaaaataaaattttcccatttataattacctgacactttcccatttccttgcctctcagtggaatacactacagtaaaatgtcatacattgagctccaataatttagaattgaaaacccagaggatggaatacagtttatcttttaaccacttacagaaaagaaatttcttaacaagcaaattcatgatgtaaaaatacaatgcaagtattttacctgcttaagggaatatacttttttcatgtacttttatttatttttatttttattttctgagatggagtttcactcttgttgcccaggctggagtgcaatggcgcgatcttggctcactgcaacctccgcctcccgagttcaagtgattctcctgcctcagcctcccgagtagctgggattacaggcatgtgccaccatgcccagctaatttttgtatgtttagtagagacggggtttcgccatgttggccaggctggtcacgaacccctgacctcaggtggtctgcctgcctcggcctcccaaattgctgggattacaggcgttagccactgcgcccagcccatgtacttttattttaaaagttaacataccaatatccataatcttgatcttggccagatgcagtggctcatggctgtaatcccagcactttgggaggctgatgtgggagaagcacttgagcttaggagttcaagaccagcctgggcagtatagtgacccccatctctaaagaaaaaaaccattagctgggcatggtggcgcatgtgagtagtcccagctacttcagaggctgaggtgggaggatagcctgagcccaggagtttgaagttatagtgaactatgatagtgccacaaaacaaaacaaataatcttgacctattcactaggaaactggactgtctatatataattgaacttaatattctataatcatgctttttgctgccttccaatttattcacattcataaattattactatttaaatttttaattagctgaagtactctattaatcagtctttatacctggctctccctagccacttaaactctgatttcttcattgatactcagggattcaatcaactttagaagtatgctagggaaaagatcagggtagcaaatcttccatataacaaattatgggggaaaagtttcatttcaaagtcaattcaatgaattttgaatcatttgctatttgttttccaggcctacaaaaatggtatcttaatcctaatgctgaaaaatgtgaccatttaagcagtttcaatgtgcttaaatttaaaaaaaaaaggcatgtaacaattatttatttgacaggtttccccaaaactgtagtcaggtaaaataaatccaatctgttatgttagtttgctactaaaggggaaaaaaaggatcaaacttacaggaaagccccacctcccctccacatgtagaaatctgtctaaagactgtctttaatgcccactatataaacaacattaaatattctaagttacaaaatagtgttaatggtttattggtaaaaatccaaactctagagtttatggaattcgtagtttggttggtatattaacactccatcttaatctttgctgctattacaaagaatgaggaaagctagaaatatctataaaaataaaataccttaaaaccgacaagcaaaatataaaagttgcatacaaattgccaataaatataaacatcacaatagaaaaattaatcttaacaaaaataaactcataattgctattaagacattataaaaacaaaaaagtttaatgtgcatgtatatttgcaaacagacacagtacactccaaacaatataattttactatcattattatataatgcagcatacaaggttactgaggtgtggtattttttgttgttgttgttgtttgcttttagtcttcttttctggaagaatgctcaccaaattcacaggaaagaagtgcctaggtgatcatttactgctatttactgcttcctggtatggagcaaaattgccctctggtaggtaactacatttctaattagtatgaaaggttctactattttcctttcttttgcttatttccccttaagcacaatttgcagaccctacttctatttaactgatcatacccttttaaatgccttgtcatcatttttcatagttcctgcatcctagaaaaaataaaaaatcatttaaaatattccttggtgtctagaaaagaaaatttctctaacaatagagattatcattttgctttctcacttaagctgatctgaatgatgatttggtactgcctttatgagcagtcctccttaataatgactaattagggccgggtgtggtggtgcatgcctgtaatcccagctacttgggaggctgaggcacgagaatcacttgaacccgggaggcggagtttgcagtaagctgagattgagccactgcactccagcctaggtgacagagcaagactttgtctcaaaaaaaaaaaaaaaaaaaaagattaattagaaaatgttgcctatgattccaggcaagttacatttccctttggacattggtactatacccataatcttgttaaaaagttaagtaggtttgctgttttatgtgcattatggatttcctccaacacagttgggaattaaaagaggtaattctactaaatattttgttttcaaatttacaaaataaatttggtgagcatttacctagatactttactgcataaaagctttccttggttcccttggacgagattcaagacaacaactaacattatttttatgaaactgtcacactcttggagttctaaaataatttatctttaaaattcttagcttcgtgctacttgaaaaataaaaatctacagcaccatcttctgaaaaggcactttctaagaaccgccttgctttaaaaaatgattaaaaaatttaactcaagagtctacgccctgacaaacgtctttgctttactgagaccctaacatagatacattagattctggttaccttagaaattagtctaaaaaaggaagggaccccgatggctggataggtgatttgacaggattctaattttgtcacaccatttacctgatacttcaacagggtttctcactggtaaatctcaaccctctatattgaatttaccatccttctatctttaattcaaattaaaatctttaacttccatattttaagaacaaaagattcttgagatttaatcaatgatgtaaacatctggagtactagttttgatgggtaaagtaatataaatttcaatgagtagtaggtaatattagcacaagccttgaccattataccttagtttaaaaaattatgttgactgacatggaaaattataaacttaaatgtaccattttaaaagtaggaaaaaagtcaaaataatttttccctttgtgtgtgtgtgtgagattatatatatacacactcatacatatacacacacacacactccccctccctgcttcctgggactcagcttggctttcactaatcacagtgtcatttctaacactgcaacggatcaagaatgttcttagtataagcaggacttttttaaaaagattttttggagaaaattctcactttctgatttctgtgctgactgacttacctactcttggctgattttttgactcctatagaatcacaaaagtgcttttctatgatcaaatatgaggactgaaataggaaaacaagagttctaaattagggttatactgctacacaggaaggcgttacttgatgtcaaacctcccaacaattcttactgaagctttaagacatttatgaattctcaaaaagaatgaaaataatgaatacttcatatggataaagccaaaataaagacgccacactaatgatatttttgcagcttgactaactaataaaaggtaatttaagtagcaagttactgttaagggcaacctgcctgttcaacagaagaacatctaagaggataagctaagcaaacatttaactcaggtttaatgatactgaatgaaaattttgcagagttgtcagttaaacttcttggtaaaaatattaaaatcaagtttgaaataggaagactgcaacatattctagctgtatcgaagtcgtttgcttcttgaatttcataaaaatcactgcccttggcaaattcatgtagggctctaaacagatccatcaagttccttgagtcacaaacggtctctaattcctggtctgcaatccatctaaatacttcggatccatcactggcatgcttagcgctcaccctttccttgaacacagagatccgctgccagtcattcctgctgaagggcaagtcaggttttatttccctagacatgccttcagtctttcatgactctgtcagaaggcctatcctcctaaaatccattagagaatacacaagcaaacactaggcagtggtgggctgtggagaagctagcttggaaactggtctagatctttagaaggctgagaatccctgtgctggaaagcagagatgcctctatcaagtgccttccaaaacactcagtaattcctactagaatccctgctagactctcttctaggaatagaaatatattaataggttataaacagggatttcccttagaatgatagtttttccaagaaacttgttagaagatcactattaagaaaaagaaagggaatctaatatttctgttgaaatgtgccaaaaaaccagtactgaagaggctgaggtaccctttttcaaactgtaaaagtcaaaatctacatttctaaaacaaagaatatcctgatattaaattgaaactaaaatggcagcaccctttgttactttgatattccgtgtccttactcttaggaaaaaaaagggtctaacactagccttgaatcctgcttatctccttactgtttagtgcagtaactgtcagaatctacttaaataaatatagcagctacaatattgtaagtgtatggtcctccatgccagtaacctgatactgtgatataatacatgtatcagcactttatgtagacacattaaccatcaagaatatacattaaactcccaactcttcttcatatgaaaatcaattatctagttgccagactgatattttacagtcagtctcgtaagatacatcacagaaaaaagaagaccaaaatctagcattcatgatatagttagtgagcaagggcaggagcagaagggtcactgtgaatttcatgtttaacttaaaaaaaaaaacttttttaaaataaaaaagattagaaattctacaccagaaatgcaacaataaataggacaaatttcaagaagcatttgtcacttagccttttatcttaaaattctaagcacaagttttcttgtaattaagaaccaatggtaattaatataccaatttgttagcaaaatagaaatatagtatacatactctttcaagttaatcaactttaaactagcaatgctgactagtgtaagagcactctaaaaaagaaatcactcaaaaggtaaagctttataatttagaaaaaatatttttcctcttaaaaaagtccttccaaatagatttaaattaagggctccactctagcatatatgagtgactgaaaattaggtgagagagtacatagagaaagggtatctacagtcattccctaaagtttcccacatgaatctgtgcagctcccatgataaaggaagatgttttactcacactgatcaagcatagacgaattaaatttttatcatcttgggtatactattttcttctcttgcccatgatcctgactatattcagtaaaatttcagtgtaaaaaaatccatctttataggaaatttttctggaggagatgggagaaggctgggagaaaaaatgtatatacgatacaaatattaccttttgtaaagttctttgcaacagtgttgtaaattgcatttcagacacttcaaaataataaacatacaaaatacagtactttcttagttttctggcagagggacaaaagatttcatgcctgtcagaggacatgggctcagattttaggctcaaaatacagtgaattggcaataatagtggattacaggtaagagagaaactaaagatctaaatccattaggtttcacgtgcagatggaattctgaaaggctaacaacaatgcccactggaaacaatctgtagtatctatactctgaaccagtgcaaaaaaaaaaaaaatcaaaatgcaattttcatgagttacaaagtgcaaagctcccctgaatccaatgttactgataaactcagttttgatagctttatagtactttttaataccttaaagtgtaatcaataaaagttttgtaaaacaatttcccacgtttcagtgatttaactgatttaaaatgatcaaagtcctaacttcctttgttactatcaccttaattttaaaaggaaagttatactggtgatacattagcaaaagttttaaaatatcatcttgcattttcctgattcattttagtaaatgaaaatgggcatctagccaatatgattcttcaataaacacaatctatttgcaaataatttaaatatgttaagctattcacaattatataaaagttcaactttatttctaatattcaagttggactcatttaggcaatttcacttcattttcattatgatttttttttcttttgagacggagttttggttttgttgcccaggctggagtgcaatggtgcagtcttggctcactgtaacttccgcctcctaggttcaagcaatcctgcctcagcctcccgagtagctgggattagaggtgcccactaccacgcccagctaatttttgtatttttagtagagacggggtttcaccacgttggccaggctggtctcaaactcctgagctccggtgatatacctgtctcagcctcccaaagtgctaggattacaggcatgagccaccgcgtccagccttttatcatgatgaattttaaaagatatgctttaaaactgaaaattacaaaactttccttctgaaattaaggctgtattctttgcccttttaaactatggaggtgcctgttcctcctactatccatggtaaagatgcagacacaactttcctttaaaactgcttattgcactaaaagatagcaaaaacaagttgtcagttcttaaaataaacatgattatatttctataaaagatgctgccaatacaattctataattattaaagcactattctaataaatataaaagaaaaggaagctatacttccaaacacatacatatgtgtttatatacacacacatacatatatatatataaaaaatatatgaaaatcacattaaggtatgagaggcagcaagtaaactatcaaaaaacaaaacaaaaaaatccctcaacaaactcttctctctactcaatttcagaggtctcaaccctacagagctctaatcttttaaaatatttaccctttataaaacctttaaagaatttccatgtataacccatagaaacagaaggcttcagaatacacatcacttaccagagagaaagttacaacttctgacaggttttatatttatagcagctttaacaaactcactaaagaaaaagaatagtaggccgggtgcggtggctcatgcctgtaatcccagcactttgggaggtcgaggcgggtggatcacaaggtcaagagatcgagaccatcctggccaacacggtgaaaccccgtctctactaaaaatacaaaaattagctgggtgtggtggcacatgcctgtaaacccagctactcgggaggctgaggcaggagaattgcttgaacccgagaggcggaagttgcagtgagccgagatctcgccactgcactccagcctggtgacagagcgaggctctgtctcattaaaaaaaaaaaagaaagaaaagaaaaagaaaaaagaaaaagaatagttcaggttgctactgcttatatacaaattgcgcaaatggtaaatgtatgttctgagtgggaggggagagacgcactctcacagaaagttattttatgtatatatatgtgtgtgtctgtgtctgtgtatgtatgtatacatatatatataaaattttgtttcttaagacagcaatatcaagagttgagaactcagaattgtgtatgagataggagtcaggagtagggtatgcaaaataaaagtagaattctagtttgccatattttatattcaaacgaaccagatacatcaacatttgaatgtcactggtaggactgggaaaaaaatgtaggtgatgaaggcaagggaaatagagaaataaaggcggtagtgggggtagaataaaagggaaagaaaattccccaatggaatgaactctaaaatatataacagacacatatatatctattatcaatccagatctagatatatatgcatatgaagtatggatgtatatattttaaaaatacacagacaccttttacaagaatatatgaatgcacattaattttttgcacacataattctgaaaaatcactttgattattcatgaaggtgtgtattttttaaaccatcatttactttttctttacttttttttgcaaagatagttgtgctgccaagcaacttgaggtaaaggcattaaaagggttagactacaagaaatgaaaacaaaacaattgcgatacttcctataggagaccgcacaaaaagcagttggctggtttcatattgcataatgatgctgtgttccttgatgaagtaaacaatcttccttgtattaacataaggatcagaccttggcccccacacagtgttggtttctgtatggctggaggtgtccttactcaattgacttcactggaaacatacgttgtatgtcaattcatctttcagtacttcctctcagagaatatacttggactatttaagcgaagtacattgtgcgtaaggtatcttggtgaatctgtacagccttggcaagagcttgtggatctcgcccattgctttgtcctgaaacgtgacttccttcagcactgtcatgttctttgtccacaagatgatatctggctctaaatgctaccaggtgagcataatacgctggtgcaggtatagaaacagatcgtgtacagcgtacgtaagtgtggcagagctggtaagttagcagctgaagttcatctgcagtaaagcagttatcatcccataaaacatgatagtgtgaaggacgactggtaccctgtattccagcatggctacagaggtaaaaatcgaactcatatgggtgtgtaatgtctgtatcaactgttgttccagctgggatattgccacttcttccaaccctttctgtcctatcagcacaaaataatcgagtgtgatgtctcttctgaactacaatgtaggttattccaggttgatagtctttctccaaactgatgcaggcttctcgaattgctagtagttcataatataatacctgcctaaactgcccctctgaaacaccatcccgataaaagatgatacgagtaggcttgaaccgagttgacttataaaattgaataagaagttcccggaccatggaggccaagtcctggatgatctcctgtcggggtctctgaactcttactgtggcacagtatctgcttgggtgtgcatccatactacctacaacagcagcaatagaaggcttctttccatcaccagcaggtggatgagtgacatcggctcccaaaaagatcactggttgctggaacacagaaggtctttgatgaggtacaagaatattattgatccctccgagtttaacatttatctttaggcacaagtttgacagagtttgaggagatgtttttattacattcttgacttgaacacattgtgtagccatacccaaaagtgtgtctcctacacgtttcacttccgcatacactggtgtcttccccggcaggatgacgataataagctgtaggccagaatatgtgttcttgagatgccggaacatgggctctacgctgtctgccccctgtgcatatttgcagaagcatggctggccctggatgggcatccctgcatccttagaaatcttacgcagctggtctgtgaaacccttcaatatttcttctctgcactgcctctgtgtggcaaaacaagcgatagcccacattttgatttcaactcctgtgtggaattgtttccctcgcatgtcccatactccatggctcggtgttgctactgtccgattccgtcctccatactggagcataggtgctggaagtacgcgtccagttacatgagccatttcatcccgaactttaaattgaaactcctgaacaaatggatctgtttcataatttgcacttcttaccaatctgctaatttcctcttgtctatctggtgcagatcttgctgttgccttgatcatagtggaagtctgattgtctgttagcttcttgatacatcgttgccctgccacaatattacagacttctagtggcaggtaggtgtgtttctgttcctgcccgacttgcagacagggaaggtgcgggtacttcagctgaagagtatacttttctctgaaatactgcgctactgttctctccacagtttggccgttttctaactgtaaaggaaaggtttgatgactggcaggcctccttgttacattacaaacacggtatttccgtctcattgttccacaatgagtcacttcaaccttcaaaccttttatctctttggtgaattttacccgatgagaatcagtcagaggtcttggttgctcatcaatattatgaatatcaagaacttcacacatgaactgaattacaggttgtgctttgtagaaggcagtggcagaaacatcgatattaagcatcattttccacatggcaggccgaacagactgatggaatccaaaccacacttccctgccccctcccagagggtggtcatatccttctggagcggagaaaaatgaacgccccacaggtgtgtatttcatggagggcagatgtcgtagcaccacatcaacggcatggacagggttagtgctgattggcttgtctaattccagtggctcaggcaaggtccgtcctgtcagtacttcatgcagtaggtgccaactcacccgagagacaaatttgattgacaccttgaaaggtcgatcttttccaccttccccaggtaaagtaacgtctaaatctacccctgtagttgccacaggaagtggattggcggtgtaaagacttctttttccatcataaactggtctacggtctccaaatatagttactttaaaatgctgaaccattgagtcaaccacctccctgttcactctcctaggacacttgtctggtttaatatctacctcatagaggtagacatcaatctttgggatttcaacttgaaaacagttagccagcagtttaatgggtttgcccatggtgccatagccaggtcttctgggcaccatgagtaggggctgggccccagcgggtcctgcggagccgatttccattcatggagctggggggagtgcttcgagggagaacggagcccgccactggcggcaaggaggcggcccggggggcgacgcggcgcgacgcgacgggcactctcactcggccccgaggcgggggcggcgacggcttcccctgagcaaccgcactccgaaagctctgggccggaagagtcgcggacggaaaacggcacaggactaggcgagaggaaggggagatgtgaggcgcggacagaggggagtcccgtccggaagttgcatcgcccgcggccgccgacgctcccaccgctcctccacgactgcgggccgccgccgccgacct

SEQ ID NO: 18657 - RNA, 15033 nt, Homo sapiens
  source 1..15033: mol_type = other RNA
tgagtgtgtgtgtgtgagtgtgtgtgatggggaaaaaagaacaattgtgtgattcacaaatggcataaaacactgattgtattacaaataagaatggtggcactctagtaagtaagataatggaatgtcaaaggaaacaaactttagaatacaaacatggaaaacatgctaaaatattaatcaagctatagcttgtggcatgtgattcttctttcccaagtattttgagagtgtcatttacccccagtagaattctatatcaactgcctctaagtccttttcctattccttcttttttttttttttgagacggagtctcactctgccacccaggctggagtgcaatggtgggatctcggctcactgcaacctccgcctcctgggttccagactaccttgtctggaaaggccctgcttggtgttttctatttaaaggggaaaaccaaacatgttatgttgatagcaatgcctggctctattaaagataaatccttcatttaatttccttattgtaattcagactagcaggattctcctgcctcagcctcaggcgcctgccaccacgcctagctaattttgtatttttagtagagacagggtttcaccatattggccacgctggtctcaaactcctgaccttgtgatccacctgccttggcctcccaaagtgctgggattgcaggcatgagccactgctcccggcctattctttcttttttaaagagggaatggggttggaccctgggctaagaaatgagaaagctcctggaaaaccttaattgcaattaattactatagaagatcaagtctgttgctagcaaaaccaaagcttccttttgttaaactccctgggatcaaactgtatccatgaactgggtcggactgtctatgccaaaattctttcttcattacaaactaaccagtgtttttaccaaatcccacaccaaaaccattttctttacaggaaagactacattgtctggaaaggccctgcttggtgttttctatttaaaggggaaaaccaaagacactatgttgatagcaatgcctggccctatttaaggataaagacttcatttaatttctttactgtaattcagaagcaacttccaagacttctctaagttactgagaataggtgtgcctttgggtctgggacaacattatcatataaatttagattacagagacgctcgtcttaggtctcttctgtaggttcaaatagcaatagctgctcttttactctgcaaatattaaacaattgtaaggtttctgtccaaggatcccagcaaggaagccttatcctaaatcccccctcactatatattctcacaatcctactagtctatttctttacaaagacctccagtttctacagattctgacaataaagagtcacgtatgcaacatttttgcagtctttccttctttggttctaaaaagactattaaaggactaacttaagagatttttgtttgttttcccaaccaaaaatgaaataaagatgaaataaagccatgaaataaagatgaaagttttgtcttttatttttaaaattattattattttttgagacggagtttcactcttgtcgcccaggctggagtgcagtggcatgatctcggctcactgcaacctccgcctaccgggttcaaacgattctctcgcctcagcctcccgagtagctgggattacaggcgcccaccaccatgcctggctaatttttgtatttttagtagagacgggttttgccatgttgtccaggctggtctcgaactcctgacctcaggtaatcagcctgcctcggcctcccgaagtgctgggattacaggtgtgagccaccgtgcccggccaagatgaaagttttaggcactaaatatcagagtaatctccctctctagtctctggtgttgcctcttcaacatcaaacataaaattatagatagcataccgccaatttttggaaagaataaaatttaaaaagcaaggctctaatgaccaacacttccatctgttttctacgcataacgctgttcatggcaattcttttttgggatgatctattactgcacaacgatttttttttttttttgagacagagtctcactctgttgcccaggctggagtgcagtggcacgatcttggctcactgcatcctccgccaccacacccggctaatttttgtatttttagaagagacagggttttgccatgttggccaggctggtcttgaactcctgacctcaggtgatctgctcacctcagctgcccaaagtgttgggattacaggtgtgagccactgcacctggccacaaagctttctttctaaagaggtgaactaaacatgaacaagccatcaagtacttcactgcggtcaagctgtactgatgtcaggtagcaggatttgtggagccaaccagttaaaacagcaaaataagctctatatgccaggtttctatgaactttcagaaggaaaaagaaaacacaggaccagaggcacctttttttgtttgtatgtttgttttgagatggagtcttgctctgttgccaggctggagtgcagcggtgcaatcttggctcactgcaacctccgcctcccaggttcaagtgattctcctgcctcagcctcccaagtagctgggactacaggcgtgtgccaccacacccagctaatttttgtatttttagtagagatggggtttcagcatgttggccaggatggtctccatctcttgacctcgtgatccgcccacctcggcctcccaaagtgcagggattacaggcgtgagccaccatgcccagcccagaggcaacttttaaaatgttggttttcaggaactacatgtctgctaaccttggacatgttgaaatgtaatgaatacaactattaaggttataagcgcaataaatatccttaaaaggggacatacaatcacagcaaaaatattttgctttttttttttttgagacggagtcttgctctgtcgcccaggctggagtgcagtggtgtgatcttggctcactgcaacctccgcctcctgggttcaagccattctcctgcctcggccttcccagtagctgggattacaggcacgtaccgccaagcccagctaatttttgtaattttagtagagacagggtttcaccatattgggcaggctggtctccaactcctgacctcgtgatccgcccgcctcagccgcccacccaaagtgctgggattacaggtgtgagctaccacgcccagccacattaatttgcttttaattagtagtaacaaattcttataatcagagtacaaatctgtactatctgtatacaattagtacttgatgtgtgcggggctgaagtatctcagaatagtatatcatagggcaaactaatgtaactggcaaaaatgcaaaaagaaatgaaatggctaatctctacaagaaatcacatgctgatctattttaaactgtaaaactttacatcatataaaaataaaattttcccatttataattacctgacactttcccatttccttgcctctcagtggaatacactacagtaaaatgtcatacattgagctccaataatttagaattgaaaacccagaggatggaatacagtttatcttttaaccacttacagaaaagaaatttcttaacaagcaaattcatgatgtaaaaatacaatgcaagtattttacctgcttaagggaatatacttttttcatgtacttttatttatttttatttttattttctgagatggagtttcactcttgttgcccaggctggagtgcaatggcgcgatcttggctcactgcaacctccgcctcccgagttcaagtgattctcctgcctcagcctcccgagtagctgggattacaggcatgtgccaccatgcccagctaatttttgtatgtttagtagagacggggtttcgccatgttggccaggctggtcacgaacccctgacctcaggtggtctgcctgcctcggcctcccaaattgctgggattacaggcgttagccactgcgcccagcccatgtacttttattttaaaagttaacataccaatatccataatcttgatcttggccagatgcagtggctcatggctgtaatcccagcactttgggaggctgatgtgggagaagcacttgagcttaggagttcaagaccagcctgggcagtatagtgacccccatctctaaagaaaaaaaccattagctgggcatggtggcgcatgtgagtagtcccagctacttcagaggctgaggtgggaggatagcctgagcccaggagtttgaagttatagtgaactatgatagtgccacaaaacaaaacaaataatcttgacctattcactaggaaactggactgtctatatataattgaacttaatattctataatcatgctttttgctgccttccaatttattcacattcataaattattactatttaaatttttaattagctgaagtactctattaatcagtctttatacctggctctccctagccacttaaactctgatttcttcattgatactcagggattcaatcaactttagaagtatgctagggaaaagatcagggtagcaaatcttccatataacaaattatgggggaaaagtttcatttcaaagtcaattcaatgaattttgaatcatttgctatttgttttccaggcctacaaaaatggtatcttaatcctaatgctgaaaaatgtgaccatttaagcagtttcaatgtgcttaaatttaaaaaaaaaaggcatgtaacaattatttatttgacaggtttccccaaaactgtagtcaggtaaaataaatccaatctgttatgttagtttgctactaaaggggaaaaaaaggatcaaacttacaggaaagccccacctcccctccacatgtagaaatctgtctaaagactgtctttaatgcccactatataaacaacattaaatattctaagttacaaaatagtgttaatggtttattggtaaaaatccaaactctagagtttatggaattcgtagtttggttggtatattaacactccatcttaatctttgctgctattacaaagaatgaggaaagctagaaatatctataaaaataaaataccttaaaaccgacaagcaaaatataaaagttgcatacaaattgccaataaatataaacatcacaatagaaaaattaatcttaacaaaaataaactcataattgctattaagacattataaaaacaaaaaagtttaatgtgcatgtatatttgcaaacagacacagtacactccaaacaatataattttactatcattattatataatgcagcatacaaggttactgaggtgtggtattttttgttgttgttgttgtttgcttttagtcttcttttctggaagaatgctcaccaaattcacaggaaagaagtgcctaggtgatcatttactgctatttactgcttcctggtatggagcaaaattgccctctggtaggtaactacatttctaattagtatgaaaggttctactattttcctttcttttgcttatttccccttaagcacaatttgcagaccctacttctatttaactgatcatacccttttaaatgccttgtcatcatttttcatagttcctgcatcctagaaaaaataaaaaatcatttaaaatattccttggtgtctagaaaagaaaatttctctaacaatagagattatcattttgctttctcacttaagctgatctgaatgatgatttggtactgcctttatgagcagtcctccttaataatgactaattagggccgggtgtggtggtgcatgcctgtaatcccagctacttgggaggctgaggcacgagaatcacttgaacccgggaggcggagtttgcagtaagctgagattgagccactgcactccagcctaggtgacagagcaagactttgtctcaaaaaaaaaaaaaaaaaaaaagattaattagaaaatgttgcctatgattccaggcaagttacatttccctttggacattggtactatacccataatcttgttaaaaagttaagtaggtttgctgttttatgtgcattatggatttcctccaacacagttgggaattaaaagaggtaattctactaaatattttgttttcaaatttacaaaataaatttggtgagcatttacctagatactttactgcataaaagctttccttggttcccttggacgagattcaagacaacaactaacattatttttatgaaactgtcacactcttggagttctaaaataatttatctttaaaattcttagcttcgtgctacttgaaaaataaaaatctacagcaccatcttctgaaaaggcactttctaagaaccgccttgctttaaaaaatgattaaaaaatttaactcaagagtctacgccctgacaaacgtctttgctttactgagaccctaacatagatacattagattctggttaccttagaaattagtctaaaaaaggaagggaccccgatggctggataggtgatttgacaggattctaattttgtcacaccatttacctgatacttcaacagggtttctcactggtaaatctcaaccctctatattgaatttaccatccttctatctttaattcaaattaaaatctttaacttccatattttaagaacaaaagattcttgagatttaatcaatgatgtaaacatctggagtactagttttgatgggtaaagtaatataaatttcaatgagtagtaggtaatattagcacaagccttgaccattataccttagtttaaaaaattatgttgactgacatggaaaattataaacttaaatgtaccattttaaaagtaggaaaaaagtcaaaataatttttccctttgtgtgtgtgtgtgagattatatatatacacactcatacatatacacacacacacactccccctccctgcttcctgggactcagcttggctttcactaatcacagtgtcatttctaacactgcaacggatcaagaatgttcttagtataagcaggacttttttaaaaagattttttggagaaaattctcactttctgatttctgtgctgactgacttacctactcttggctgattttttgactcctatagaatcacaaaagtgcttttctatgatcaaatatgaggactgaaataggaaaacaagagttctaaattagggttatactgctacacaggaaggcgttacttgatgtcaaacctcccaacaattcttactgaagctttaagacatttatgaattctcaaaaagaatgaaaataatgaatacttcatatggataaagccaaaataaagacgccacactaatgatatttttgcagcttgactaactaataaaaggtaatttaagtagcaagttactgttaagggcaacctgcctgttcaacagaagaacatctaagaggataagctaagcaaacatttaactcaggtttaatgatactgaatgaaaattttgcagagttgtcagttaaacttcttggtaaaaatattaaaatcaagtttgaaataggaagactgcaacatattctagctgtatcgaagtcgtttgcttcttgaatttcataaaaatcactgcccttggcaaattcatgtagggctctaaacagatccatcaagttccttgagtcacaaacggtctctaattcctggtctgcaatccatctaaatacttcggatccatcactggcatgcttagcgctcaccctttccttgaacacagagatccgctgccagtcattcctgctgaagggcaagtcaggttttatttccctagacatgccttcagtctttcatgactctgtcagaaggcctatcctcctaaaatccattagagaatacacaagcaaacactaggcagtggtgggctgtggagaagctagcttggaaactggtctagatctttagaaggctgagaatccctgtgctggaaagcagagatgcctctatcaagtgccttccaaaacactcagtaattcctactagaatccctgctagactctcttctaggaatagaaatatattaataggttataaacagggatttcccttagaatgatagtttttccaagaaacttgttagaagatcactattaagaaaaagaaagggaatctaatatttctgttgaaatgtgccaaaaaaccagtactgaagaggctgaggtaccctttttcaaactgtaaaagtcaaaatctacatttctaaaacaaagaatatcctgatattaaattgaaactaaaatggcagcaccctttgttactttgatattccgtgtccttactcttaggaaaaaaaagggtctaacactagccttgaatcctgcttatctccttactgtttagtgcagtaactgtcagaatctacttaaataaatatagcagctacaatattgtaagtgtatggtcctccatgccagtaacctgatactgtgatataatacatgtatcagcactttatgtagacacattaaccatcaagaatatacattaaactcccaactcttcttcatatgaaaatcaattatctagttgccagactgatattttacagtcagtctcgtaagatacatcacagaaaaaagaagaccaaaatctagcattcatgatatagttagtgagcaagggcaggagcagaagggtcactgtgaatttcatgtttaacttaaaaaaaaaaacttttttaaaataaaaaagattagaaattctacaccagaaatgcaacaataaataggacaaatttcaagaagcatttgtcacttagccttttatcttaaaattctaagcacaagttttcttgtaattaagaaccaatggtaattaatataccaatttgttagcaaaatagaaatatagtatacatactctttcaagttaatcaactttaaactagcaatgctgactagtgtaagagcactctaaaaaagaaatcactcaaaaggtaaagctttataatttagaaaaaatatttttcctcttaaaaaagtccttccaaatagatttaaattaagggctccactctagcatatatgagtgactgaaaattaggtgagagagtacatagagaaagggtatctacagtcattccctaaagtttcccacatgaatctgtgcagctcccatgataaaggaagatgttttactcacactgatcaagcatagacgaattaaatttttatcatcttgggtatactattttcttctcttgcccatgatcctgactatattcagtaaaatttcagtgtaaaaaaatccatctttataggaaatttttctggaggagatgggagaaggctgggagaaaaaatgtatatacgatacaaatattaccttttgtaaagttctttgcaacagtgttgtaaattgcatttcagacacttcaaaataataaacatacaaaatacagtactttcttagttttctggcagagggacaaaagatttcatgcctgtcagaggacatgggctcagattttaggctcaaaatacagtgaattggcaataatagtggattacaggtaagagagaaactaaagatctaaatccattaggtttcacgtgcagatggaattctgaaaggctaacaacaatgcccactggaaacaatctgtagtatctatactctgaaccagtgcaaaaaaaaaaaaaatcaaaatgcaattttcatgagttacaaagtgcaaagctcccctgaatccaatgttactgataaactcagttttgatagctttatagtactttttaataccttaaagtgtaatcaataaaagttttgtaaaacaatttcccacgtttcagtgatttaactgatttaaaatgatcaaagtcctaacttcctttgttactatcaccttaattttaaaaggaaagttatactggtgatacattagcaaaagttttaaaatatcatcttgcattttcctgattcattttagtaaatgaaaatgggcatctagccaatatgattcttcaataaacacaatctatttgcaaataatttaaatatgttaagctattcacaattatataaaagttcaactttatttctaatattcaagttggactcatttaggcaatttcacttcattttcattatgatttttttttcttttgagacggagttttggttttgttgcccaggctggagtgcaatggtgcagtcttggctcactgtaacttccgcctcctaggttcaagcaatcctgcctcagcctcccgagtagctgggattagaggtgcccactaccacgcccagctaatttttgtatttttagtagagacggggtttcaccacgttggccaggctggtctcaaactcctgagctccggtgatatacctgtctcagcctcccaaagtgctaggattacaggcatgagccaccgcgtccagccttttatcatgatgaattttaaaagatatgctttaaaactgaaaattacaaaactttccttctgaaattaaggctgtattctttgcccttttaaactatggaggtgcctgttcctcctactatccatggtaaagatgcagacacaactttcctttaaaactgcttattgcactaaaagatagcaaaaacaagttgtcagttcttaaaataaacatgattatatttctataaaagatgctgccaatacaattctataattattaaagcactattctaataaatataaaagaaaaggaagctatacttccaaacacatacatatgtgtttatatacacacacatacatatatatatataaaaaatatatgaaaatcacattaaggtatgagaggcagcaagtaaactatcaaaaaacaaaacaaaaaaatccctcaacaaactcttctctctactcaatttcagaggtctcaaccctacagagctctaatcttttaaaatatttaccctttataaaacctttaaagaatttccatgtataacccatagaaacagaaggcttcagaatacacatcacttaccagagagaaagttacaacttctgacaggttttatatttatagcagctttaacaaactcactaaagaaaaagaatagtaggccgggtgcggtggctcatgcctgtaatcccagcactttgggaggtcgaggcgggtggatcacaaggtcaagagatcgagaccatcctggccaacacggtgaaaccccgtctctactaaaaatacaaaaattagctgggtgtggtggcacatgcctgtaaacccagctactcgggaggctgaggcaggagaattgcttgaacccgagaggcggaagttgcagtgagccgagatctcgccactgcactccagcctggtgacagagcgaggctctgtctcattaaaaaaaaaaaagaaagaaaagaaaaagaaaaaagaaaaagaatagttcaggttgctactgcttatatacaaattgcgcaaatggtaaatgtatgttctgagtgggaggggagagacgcactctcacagaaagttattttatgtatatatatgtgtgtgtctgtgtctgtgtatgtatgtatacatatatatataaaattttgtttcttaagacagcaatatcaagagttgagaactcagaattgtgtatgagataggagtcaggagtagggtatgcaaaataaaagtagaattctagtttgccatattttatattcaaacgaaccagatacatcaacatttgaatgtcactggtaggactgggaaaaaaatgtaggtgatgaaggcaagggaaatagagaaataaaggcggtagtgggggtagaataaaagggaaagaaaattccccaatggaatgaactctaaaatatataacagacacatatatatctattatcaatccagatctagatatatatgcatatgaagtatggatgtatatattttaaaaatacacagacaccttttacaagaatatatgaatgcacattaattttttgcacacataattctgaaaaatcactttgattattcatgaaggtgtgtattttttaaaccatcatttactttttctttacttttttttgcaaagatagttgtgctgccaagcaacttgaggtaaaggcattaaaagggttagactacaagaaatgaaaacaaaacaattgcgatacttcctataggagaccgcacaaaaagcagttggctggtttcatattgcataatgatgctgtgttccttgatgaagtaaacaatcttccttgtattaacataaggatcagaccttggcccccacacagtgttggtttctgtatggctggaggtgtccttactcaattgacttcactggaaacatacgttgtatgtcaattcatctttcagtacttcctctcagagaatatacttggactatttaagcgaagtacattgtgcgtaaggtatcttggtgaatctgtacagccttggcaagagcttgtggatctcgcccattgctttgtcctgaaacgtgacttccttcagcactgtcatgttctttgtccacaagatgatatctggctctaaatgctaccaggtgagcataatacgctggtgcaggtatagaaacagatcgtgtacagcgtacgtaagtgtggcagagctggtaagttagcagctgaagttcatctgcagtaaagcagttatcatcccataaaacatgatagtgtgaaggacgactggtaccctgtattccagcatggctacagaggtaaaaatcgaactcatatgggtgtgtaatgtctgtatcaactgttgttccagctgggatattgccacttcttccaaccctttctgtcctatcagcacaaaataatcgagtgtgatgtctcttctgaactacaatgtaggttattccaggttgatagtctttctccaaactgatgcaggcttctcgaattgctagtagttcataatataatacctgcctaaactgcccctctgaaacaccatcccgataaaagatgatacgagtaggcttgaaccgagttgacttataaaattgaataagaagttcccggaccatggaggccaagtcctggatgatctcctgtcggggtctctgaactcttactgtggcacagtatctgcttgggtgtgcatccatactacctacaacagcagcaatagaaggcttctttccatcaccagcaggtggatgagtgacatcggctcccaaaaagatcactggttgctggaacacagaaggtctttgatgaggtacaagaatattattgatccctccgagtttaacatttatctttaggcacaagtttgacagagtttgaggagatgtttttattacattcttgacttgaacacattgtgtagccatacccaaaagtgtgtctcctacacgtttcacttccgcatacactggtgtcttccccggcaggatgacgataataagctgtaggccagaatatgtgttcttgagatgccggaacatgggctctacgctgtctgccccctgtgcatatttgcagaagcatggctggccctggatgggcatccctgcatccttagaaatcttacgcagctggtctgtgaaacccttcaatatttcttctctgcactgcctctgtgtggcaaaacaagcgatagcccacattttgatttcaactcctgtgtggaattgtttccctcgcatgtcccatactccatggctcggtgttgctactgtccgattccgtcctccatactggagcataggtgctggaagtacgcgtccagttacatgagccatttcatcccgaactttaaattgaaactcctgaacaaatggatctgtttcataatttgcacttcttaccaatctgctaatttcctcttgtctatctggtgcagatcttgctgttgccttgatcatagtggaagtctgattgtctgttagcttcttgatacatcgttgccctgccacaatattacagacttctagtggcaggtaggtgtgtttctgttcctgcccgacttgcagacagggaaggtgcgggtacttcagctgaagagtatacttttctctgaaatactgcgctactgttctctccacagtttggccgttttctaactgtaaaggaaaggtttgatgactggcaggcctccttgttacattacaaacacggtatttccgtctcattgttccacaatgagtcacttcaaccttcaaaccttttatctctttggtgaattttacccgatgagaatcagtcagaggtcttggttgctcatcaatattatgaatatcaagaacttcacacatgaactgaattacaggttgtgctttgtagaaggcagtggcagaaattcatggagggcagatgtcgtagcaccacatcaacggcatggacagggttagtgctgattggcttgtctaattccagtggctcaggcaaggtccgtcctgtcagtacttcatgcagtaggtgccaactcacccgagagacaaatttgattgacaccttgaaaggtcgatcttttccaccttccccaggtaaagtaacgtctaaatctacctgttcactctcctaggacacttgtctggtttaatatctacctcatagaggtagacatcaatctttgggatttcaacttgaaaacagttagccagcagtttaatgggtttgcccatggtgccatagccaggtcttctgggcaccatgagtaggggctgggccccagcgggtcctgcggagccgatttccattcatggagctggggggagtgcttcgagggagaacggagcccgccactggcggcaaggaggcggcccggggggcgacgcggcgcgacgcgacgggcactctcactcggccccgaggcgggggcggcgacggcttcccctgagcaaccgcactccgaaagctctgggccggaagagtcgcggacggaaaacggcacaggactaggcgagaggaaggggagatgtgaggcgcggacagaggggagtcccgtccggaagttgcatcgcccgcggccgccgacgctcccaccgctcctccacgactgcgggccgccgccgccgacct

SEQ ID NO: 18658 - RNA, 1579 nt, Homo sapiens
  source 1..1579: mol_type = other RNA
tgagtgtgtgtgtgtgagtgtgtgtgtatatatatatttcaatcctcacaataacgctaggagatcagtgctctgcttatatcatcttagagatggcaaaactcatgaagagttaatttaaataactttccaaatttacaaagctaggaaaaggtggagctcagattcaaacccagcaaatctggcaccagcctcttcagagactaaattgatcaagttgtggtaaaactcccagagttgcaaggcatagccttatctatttgtccctatatttttttgcttgattcccaaagtgctagagtgggcatccttctggaagctgagggtcaccaatatagaatcttaaggggacatttttggttttctaaaagaagcaaattgcaattttaggaaaagtatagtttagacatactaaaagtatttaagaaaatattggattttgctgtttctttgtgactatttttgttgttgctgttcctctacattctattttatctacaatagagatctttaagaaaaaaaaaagtacttgccttcaagggcaggtgatgccggagtgggtctggaagcttgttctgtcggtaagggaggtggaatggctgggctttgtcctttctgttcatgctttgacacagctgctttctctttgtcctccttttctttgggttttgatggtgttttctgtacttcttttacttttgcagctgtttgcttcactttctcctgttttccacctttcacttcctttttagtcttttcttcactcttttctgcagtcttagctttcttctgttctttcgccagtgtctttgtttctggtttttcttttttctcaattttttccttgtgagttgctttcttttcaggtttttctttttctcttactttttcttttcctttttctttttctttgtgtgtaactttagtttgtattttcctttcaggtttctcttgtttttcagtcttatctttgtgtatttctttttttctcaagggaggctcatctatttctcctttatcagtatcttcgtcaccatcatcatcttcttcatcttcagatgagatgatgtcagataacaaagaaaagaagccatagatccagtccgtggtttcctccatagcatcacgtaccagttttaaaggatctgagccaatcttggcaatagagcttgctgaaaagtttttgtaatccactaaatcaaacataacgatggcaacagctgaccacgtgattatcagggcaatgaccagaagccaggctgcaggggagctgaacgtcgtcactatgtcttctgtgactgtcctcttcagcacttttccgggggatttgggcacagatccatttttgctgtctatcacagttgtggttgtagatgcatttccttcagcagtgatctcagtcatggtggtcgtcaaaagtaaaagtcagttgaaaagttcccgtcaagttgcactttgcagagtatttggggatttgagaactctggtggagggttctgtgtcaaaacctgggggctcttcgttttcctggctgtttctgctgcttctttgttgtcctgttgaactttgcctctcctct

SEQ ID NO: 18659 - RNA, 3474 nt, Homo sapiens
  source 1..3474: mol_type = other RNA
tgagtgtgtgtgtgtgagtgtgtgtgtatattttgtagcatttgaagttttgtggcaagatttctatcaaattgaatgttgtcttgtttcctatggtgggtgagacccaaggtgccagtgtttgaagtaatcattcagattggagtagcattttttcatgtgttactatattttccattcctttccagtcaacccagtaagataaatgctatttcaggggatatggtatctacaaaatttttcatttggatgtgtttgtatttgctaagtacaaatctacaccaatattgtcacttgtatattgtaccaacatatggcaggaaagcctggctggtcacaccaagtcttatttttcatcttgggatacgagttgccaacgatctgatatgacttgaaaaacaaacagacaaatctgcatcactaaaaaggcttatgtttctttaaaacatttcaaataaataattcatattaacgaaaaccgtccagccaagtcgaatactttgctgattgctatatttaattattgctaacaaattctgagcaggctgttttccagcatcctgtgcttttgtgagtgcggattccccactagtgggcgccatttgtcttcttattccttccgtgcagctcaccttaccgcaaattcatttataaatacaaaaatcagtgaaaggtgggggaagaagtgtgcaataaaaatcaaactcaactatagtgcagtccttagacaaggatttccttcaccctttcctgtttcctcattaaaacccagcaagaaagatgacttgagaatagcatttctatttaaatcctattggaaaataaattaataaacacacttgtaaaaatacggcagacttcaaaatgcagttaaaagataaaaaactctttgattagtaataaataaattataaaaatgtcacatttattttacatatactttacaaaaaaaaaaagagtacaatgaagaaataaaagaaaaacatatgaaaataaataagatctaataattgactgcattgcttttaatccaagaagtctatcatagtttttctttcctttttatatcagctggggaaaataaaattagtgcaatgttgcaaattgtaaatgcagtacggcaacctccacgccttagcagtacatgaacctctaacagatccatctggagtttactgctgttggtaacttctgttgcccggcagcgctgtgatcctacacatggatacccttcactgcctgtttgatactttccagtagagctttgcattccggggaatagtcccgttccagattgctgtacatatctgtgagtgtatttacatatgcttcaaaattctgctcactgataggtcccatctgtggaagctggatgtcagcaaggcttgaaatgagagcttggcttagacctgccagctctttcagcagactttcattgttctgttctatgagtttgttctcctcctctatcgtctttaagttgctctccatagatgtgatctgggtctgaagtttcatcatatctgcttcaattttaaggttggattcattcagttcctttatttcttcatccaaatgcctaatttcttcatcactctctattcccccagttgctttgagcttgatggtcatgagttcttcagaaaccttgccctttttgataacttgtgcattgagaggacatccagataagcttcggtgggtgacaaaaacattatttacatggcccagcccattgcagcctggcaagggacaatgtggtagctcttgtttgttcagtttccaggagagggaggctccattgagaggattctccttctgtctcttggcagccagaggacagccagaagctgtgcggtgtgatgtgtatttacctgatatgtgaccttggccatcacaccctatcacaggacatttcagttcagggtcttctttttcttccttggtaggggtcattttgacaccacctttccttgcacgagggcatccggacaagcttctgtgggaagcatagtttccagtcacgtgccccgagccatcgcagcctggggttggacacttaagctcctgagagttggcagccatgagggattttagagtcttatctgctaaaggacatccagaaacactgcgatgagatgcatagtttcctgtcacgtggccacttccatcacatcctggtgttggacaggtgattagttcctttttgagatctcttgcatgaagcttgggtttagggcttggtatagaggcctctccaggaaactttttttcctctaaattttctagagagctcactgggtctttctctttctcctcctctgtcttcccgtgagttttgctatagttgataggagtgtcccagccctcttggtcacaaagagcctgatagaatgctgcattgaccagaatgctgcttgttttgaatggggaagaggaaggagttggaatagaagtgttagaggaagttaggggtgcagacttgtccaggattcgattttttttcatgcttaagtccaatgtgccattttcatccacttctatttcggctcccttggcatgcagactctgtggcttgttggagaggatgtctgtggcttccctgcagcgggtggaaaggttcaggatggcagcagctgctgctatgtgggtgtcttcactacattgaccgtagctataagagctggcacggccagggctctgggtgtgggcgcctgcactaggcagtcgattaggaaatttcactggatttggaaaatgctttgattcaggaaatggtggtgtttttcgtccttgcactgtttgtatgagagggcgtttaccgaaaacttgggcatcaaaactggcataatcaaatggtacttttccaaacttctcttgttcttttgacactgtggctctgggagaggtgatggcttgtgacgggaaattgaattcaatttgcttcaccaaacttgtcctgtgggcctggtcaggacactgcccagtttggggagaatcaagctgatttttatcctgggacattgccaatttttcagctgcagcaattggacaaccagaaagactcctgtgggtgttgcggttgctgttcacatgaccccttcctgtgcatcccggcgtgggacacttgagcacattttcatgcatggcaagaatttccaggggaacccgcactttgtgggggcaccccgaaaggctgcggtggtgcgggtagagccctgtcacgtgtcccgtgccatcacatccagggatcgggcacttggtctccctcttttcaggccttggtgaatcttttttcatgtgtgaaaatagtccaaaattaacacagcttgattggaggataatctagagagtgggggaaaagaaagaaattgtttattttataattataaattgatttttaagttgcattaaactgttaaaaagctacctgaaaaaaataatcaaatctgacttttttttcaaaccctaatg

SEQ ID NO: 18660 - RNA, 5087 nt, Homo sapiens
  source 1..5087: mol_type = other RNA
tgagtgtgtgtgtgtgagtgtgtgtgtatattttgtagcatttgaagttttgtggcaagatttctatcaaattgaatgttgtcttgtttcctatggtgggtgagacccaaggtgccagtgtttgaagtaatcattcagattggagtagcattttttcatgtgttactatattttccattcctttccagtcaacccagtaagataaatgctatttcaggggatatggtatctacaaaatttttcatttggatgtgtttgtatttgctaagtacaaatctacaccaatattgtcacttgtatattgtaccaacatatggcaggaaagcctggctggtcacaccaagtcttatttttcatcttgggatacgagttgccaacgatctgatatgacttgaaaaacaaacagacaaatctgcatcactaaaaaggcttatgtttctttaaaacatttcaaataaataattcatattaacgaaaaccgtccagccaagtcgaatactttgctgattgctatatttaattattgctaacaaattctgagcaggctgttttccagcatcctgtgcttttgtgagtgcggattccccactagtgggcgccatttgtcttcttattccttccgtgcagctcaccttaccgcaaattcatttataaatacaaaaatcagtgaaaggtgggggaagaagtgtgcaataaaaatcaaactcaactatagtgcagtccttagacaaggatttccttcaccctttcctgtttcctcattaaaacccagcaagaaagatgacttgagaatagcatttctatttaaatcctattggaaaataaattaataaacacacttgtaaaaatacggcagacttcaaaatgcagttaaaagataaaaaactctttgattagtaataaataaattataaaaatgtcacatttattttacatatactttacaaaaaaaaaaagagtacaatgaagaaataaaagaaaaacatatgaaaataaataagatctaataattgactgcattgcttttaatccaagaagtctatcatagtttttctttcctttttatatcagctggggaaaataaaattagtgcaatgttgcaaattgtaaatgcagtacggcaacctccacgccttagcagtacatgaacctctaacagatccatctggagtttactgctgttggtaacttctgttgcccggcagcgctgtgatcctacacatggatacccttcactgcctgtttgatactttccagtagagctttgcattccggggaatagtcccgttccagattgctgtacatatctgtgagtgtatttacatatgcttcaaaattctgctcactgataggtcccatctgtggaagctggatgtcagcaaggcttgaaatgagagcttggcttagacctgccagctctttcagcagactttcattgttctgttctatgagtttgttctcctcctctatcgtctttaagttgctctccatagatgtgatctgggtctgaagtttcatcatatctgcttcaattttaaggttggattcattcagttcctttatttcttcatccaaatgcctaatttcttcatcactctctattcccccagttgctttgagcttgatggtcatgagttcttcagaaaccttgccctttttgataacttgtgcattgagaggacatccagataagcttcggtgggtgacaaaaacattatttacatggcccagcccattgcagcctggcaagggacaatgtggtagctcttgtttgttcagtttccaggagagggaggctccattgagaggattctccttctgtctcttggcagccagaggacagccagaagctgtgcggtgtgatgtgtatttacctgatatgtgaccttggccatcacaccctatcacaggacatttcagttcagggtcttctttttcttccttggtaggggtcattttgacaccacctttccttgcacgagggcatccggacaagcttctgtgggaagcatagtttccagtcacgtgccccgagccatcgcagcctggggttggacacttaagctcctgagagttggcagccatgagggattttagagtcttatctgctaaaggacatccagaaacactgcgatgagatgcatagtttcctgtcacgtggccacttccatcacatcctggtgttggacaggtgattagttcctttttgagatctcttgcatgaagcttgggtttagggcttggtatagaggcctctccaggaaactttttttcctctaaattttctagagagctcactgggtctttctctttctcctcctctgtcttcccgtgagttttgctatagttgataggagtgtcccagccctcttggtcacaaagagcctgatagaatgctgcattgaccagaatgctgcttgttttgaatggggaagaggaaggagttggaatagaagtgttagaggaagttaggggtgcagacttgtccaggattcgattttttttcatgcttaagtccaatgtgccattttcatccacttctatttcggctcccttggcatgcagactctgtggcttgttggagaggatgtctgtggcttccctgcagcgggtggaaaggttcaggatggcagcagctgctgctatgtgggtgtcttcactacattgaccgtagctataagagctggcacggccagggctctgggtgtgggcgcctgcactaggcagtcgattaggaaatttcactggatttggaaaatgctttgattcaggaaatggtggtgtttttcgtccttgcactgtttgtatgagagggcgtttaccgaaaacttgggcatcaaaactggcataatcaaatggtacttttccaaacttctcttgttcttttgacactgtggctctgggagaggtgatggcttgtgacgggaaattgaattcaatttgcttcaccaaacttgtcctgtgggcctggtcaggacactgcccagtttggggagaatcaagctgatttttatcctgggacattgccaatttttcagctgcagcaattggacaaccagaaagactcctgtgggtgttgcggttgctgttcacatgaccccttcctgtgcatcccggcgtgggacacttgagcacattttcatgcatggcaagaatttccaggggaacccgcactttgtgggggcaccccgaaaggctgcggtggtgcgggtagagccctgtcacgtgtcccgtgccatcacatccagggatcgggcacttggtctccctcttttcaggccttggtgaatcttttttcatgtgtgaaaatagtccaaaattaacacagcttgattggaggataatgtttattgttaaagatttgtcttccacccatgtcgataactttggtttgcctcctttcccctgctaggtgctccagcaggaacctatccagctctttgtaggtgttatggaaaacacaacctcgctcagcctgcagagcaattgcctgctccagcaaacttaaattccccttggccttttccaggtcactaccctcttccgtcattactgccaggctctcgctatcttcctcctcaacgtcagggaatgagggctgggcattgccatccaggggttctgcgagagcattctgcgggtctttcctttctgtttcagaatcacacctgttctcacaagggataaatttgtcaccttcagtttttatttcaggaacttccaataggtcttttttatgatctgttaaaacatactttgggactctaggtggtttggtttcttctgagaagttggagccactgtcccagccattttctgcactttcagagttactttcattgtcatcagaggagcagaagggtggctgagaatcatcaatcttgtctcttccatcatcagaatgaatcagaaagcactcgtctgcttcatcgctctctgcttttaaagactggatgccactgtcatttaaattttcacttacagtctgaacagatacatttttttcaaatttccccaagtgcattaaagacttgaccatgagctcttgataacaagagtatctgtcttccttcctactggagttttcttgtgcagttgaaagaagactttcatccataggttttatcatgatttcctctgcggtagagtgaccatgtgtttccaaggggccatcgtcctctgtcctgtcactgcggtcttcttggcagtctgcttttgggctgtagtgtcggggcttcattagcagggatttccttttgttgactggaacccccaaagcctgatcttcagctgttctcttctttgccatggagcaatcataggcaacactgagctcctggattagtgaatccattggcacctcggttcctttagagcgagtacgcagcgttttatcttcagcctctgcatccatctataaacagatgtataaagtgatttcctagtacttgtacttgacgtcttttcttactggagcttacatcaggggcaataagcaggtctcttccacatcgccccagtgcacagatctggtaccttcttttaggctgaagaggaagtcctggaattgctctctttttctccaggtaacttgtatgtcaactcagtttgccctgctgtgtcagggggactaaataaatgactttgtcttatttagtgataaatcctgaaattcattctttcttgcagaaaatttctaccgtcctgccttctctaccctttgcagtatatcaaagtgctcagctttttaatcatagatttctgtgtttcttgtaggatttgaccagacattaaatagatgcttcttcaacttaagtcagcaactgtagttccttccctaaaagctactggatctgaactggagagtttccatcactccttagtcttgatatgagcacgcagacacataaaatggaattgtcacaatgcttcagggacactcacaaaattgggggctcggtgcctcctagcctttgttctgcctctcacgctgacatcagggaagcagtgatgtagaataaagcaggggtgggctaggttagtccagtgtttgtgtcgttgtgtggtgtgcagggacactctgtgat

SEQ ID NO: 18661 - RNA, 5245 nt, Homo sapiens
  source 1..5245: mol_type = other RNA
tgagtgtgtgtgtgtgagtgtgtgtgtatattttgtagcatttgaagttttgtggcaagatttctatcaaattgaatgttgtcttgtttcctatggtgggtgagacccaaggtgccagtgtttgaagtaatcattcagattggagtagcattttttcatgtgttactatattttccattcctttccagtcaacccagtaagataaatgctatttcaggggatatggtatctacaaaatttttcatttggatgtgtttgtatttgctaagtacaaatctacaccaatattgtcacttgtatattgtaccaacatatggcaggaaagcctggctggtcacaccaagtcttatttttcatcttgggatacgagttgccaacgatctgatatgacttgaaaaacaaacagacaaatctgcatcactaaaaaggcttatgtttctttaaaacatttcaaataaataattcatattaacgaaaaccgtccagccaagtcgaatactttgctgattgctatatttaattattgctaacaaattctgagcaggctgttttccagcatcctgtgcttttgtgagtgcggattccccactagtgggcgccatttgtcttcttattccttccgtgcagctcaccttaccgcaaattcatttataaatacaaaaatcagtgaaaggtgggggaagaagtgtgcaataaaaatcaaactcaactatagtgcagtccttagacaaggatttccttcaccctttcctgtttcctcattaaaacccagcaagaaagatgacttgagaatagcatttctatttaaatcctattggaaaataaattaataaacacacttgtaaaaatacggcagacttcaaaatgcagttaaaagataaaaaactctttgattagtaataaataaattataaaaatgtcacatttattttacatatactttacaaaaaaaaaaagagtacaatgaagaaataaaagaaaaacatatgaaaataaataagatctaataattgactgcattgcttttaatccaagaagtctatcatagtttttctttcctttttatatcagctggggaaaataaaattagtgcaatgttgcaaattgtaaatgcagtacggcaacctccacgccttagcagtacatgaacctctaacagatccatctggagtttactgctgttggtaacttctgttgcccggcagcgctgtgatcctacacatggatacccttcactgcctgtttgatactttccagtagagctttgcattccggggaatagtcccgttccagattgctgtacatatctgtgagtgtatttacatatgcttcaaaattctgctcactgataggtcccatctgtggaagctggatgtcagcaaggcttgaaatgagagcttggcttagacctgccagctctttcagcagactttcattgttctgttctatgagtttgttctcctcctctatcgtctttaagttgctctccatagatgtgatctgggtctgaagtttcatcatatctgcttcaattttaaggttggattcattcagttcctttatttcttcatccaaatgcctaatttcttcatcactctctattcccccagttgctttgagcttgatggtcatgagttcttcagaaaccttgccctttttgataacttgtgcattgagaggacatccagataagcttcggtgggtgacaaaaacattatttacatggcccagcccattgcagcctggcaagggacaatgtggtagctcttgtttgttcagtttccaggagagggaggctccattgagaggattctccttctgtctcttggcagccagaggacagccagaagctgtgcggtgtgatgtgtatttacctgatatgtgaccttggccatcacaccctatcacaggacatttcagttcagggtcttctttttcttccttggtaggggtcattttgacaccacctttccttgcacgagggcatccggacaagcttctgtgggaagcatagtttccagtcacgtgccccgagccatcgcagcctggggttggacacttaagctcctgagagttggcagccatgagggattttagagtcttatctgctaaaggacatccagaaacactgcgatgagatgcatagtttcctgtcacgtggccacttccatcacatcctggtgttggacaggtgattagttcctttttgagatctcttgcatgaagcttgggtttagggcttggtatagaggcctctccaggaaactttttttcctctaaattttctagagagctcactgggtctttctctttctcctcctctgtcttcccgtgagttttgctatagttgataggagtgtcccagccctcttggtcacaaagagcctgatagaatgctgcattgaccagaatgctgcttgttttgaatggggaagaggaaggagttggaatagaagtgttagaggaagttaggggtgcagacttgtccaggattcgattttttttcatgcttaagtccaatgtgccattttcatccacttctatttcggctcccttggcatgcagactctgtggcttgttggagaggatgtctgtggcttccctgcagcgggtggaaaggttcaggatggcagcagctgctgctatgtgggtgtcttcactacattgaccgtagctataagagctggcacggccagggctctgggtgtgggcgcctgcactaggcagtcgattaggaaatttcactggatttggaaaatgctttgattcaggaaatggtggtgtttttcgtccttgcactgtttgtatgagagggcgtttaccgaaaacttgggcatcaaaactggcataatcaaatggtacttttccaaacttctcttgttcttttgacactgtggctctgggagaggtgatggcttgtgacgggaaattgaattcaatttgcttcaccaaacttgtcctgtgggcctggtcaggacactgcccagtttggggagaatcaagctgatttttatcctgggacattgccaatttttcagctgcagcaattggacaaccagaaagactcctgtgggtgttgcggttgctgttcacatgaccccttcctgtgcatcccggcgtgggacacttgagcacattttcatgcatggcaagaatttccaggggaacccgcactttgtgggggcaccccgaaaggctgcggtggtgcgggtagagccctgtcacgtgtcccgtgccatcacatccagggatcgggcacttggtctccctcttttcaggccttggtgaatcttttttcatgtgtgaaaatagtccaaaattaacacagcttgattggaggataatgtttattgttaaagatttgtcttccacccatgtcgataactttggtttgcctcctttcccctgctaggtgctccagcaggaacctatccagctctttgtaggtgttatggaaaacacaacctcgctcagcctgcagagcaattgcctgctccagcaaacttaaattccccttggccttttccaggtcactaccctcttccgtcattactgccaggctctcgctatcttcctcctcaacgtcagggaatgagggctgggcattgccatccaggggttctgcgagagcattctgcgggtctttcctttctgtttcagaatcacacctgttctcacaagggataaatttgtcaccttcagtttttatttcaggaacttccaataggtcttttttatgatctgttaaaacatactttgggactctaggtggtttggtttcttctgagaagttggagccactgtcccagccattttctgcactttcagagttactttcattgtcatcagaggagcagaagggtggctgagaatcatcaatcttgtctcttccatcatcagaatgaatcagaaagcactcgtctgcttcatcgctctctgcttttaaagactggatgccactgtcatttaaattttcacttacagtctgaacagatacatttttttcaaatttccccaagtgcattaaagacttgaccatgagctcttgataacaagagtatctgtcttccttcctactggagttttcttgtgcagttgaaagaagactttcatccataggttttatcatgatttcctctgcggtagagtgaccatgtgtttccaaggggccatcgtcctctgtcctgtcactgcggtcttcttggcagtctgcttttgggctgtagtgtcggggcttcattagcagggatttccttttgttgactggaacccccaaagcctgatcttcagctgttctcttctttgccatggagcaatcataggcaacactttttttctctgaatgacttggttcctttaaaggactctggtgtccctcaccaggtaagtggcctcatgtccacgggcacactgattctgagctcctggattagtgaatccattggcacctcggttcctttagagcgagtacgcagcgttttatcttcagcctctgcatccatctataaacagatgtataaagtgatttcctagtacttgtacttgacgtcttttcttactggagcttacatcaggggcaataagcaggtctcttccacatcgccccagtgcacagatctggtaccttcttttaggctgaagaggaagtcctggaattgctctctttttctccaggtaacttgtatgtcaactcagtttgccctgctgtgtcagggggactaaataaatgactttgtcttatttagtgataaatcctgaaattcattctttcttgcagaaaatttctaccgtcctgccttctctaccctttgcagtatatcaaagtgctcagctttttaatcatagatttctgtgtttcttgtaggatttgaccagacattaaatagatgcttcttcaacttaagtcagcaactgtagttccttccctaaaagctactggatctgaactggagagtttccatcactccttagtcttgatatgagcacgcagacacataaaatggaattgtcacaatgcttcagggacactcacaaaattgggggctctttacctggcgaacgtctacaggtgtgtcgaaagttatcttttcctggatgtgttccaaaatgctcttatgctatttctcttaggatttctccacgctgccccattcagaaattttattattttctctagtattcccctgaggtcacattcagttaaaaacatcctgcccttctccctacaaaaaggttccatagaatc

SEQ ID NO: 18662 - RNA, 5136 nt, Homo sapiens
  source 1..5136: mol_type = other RNA
tgagtgtgtgtgtgtgagtgtgtgtgtatattttgtagcatttgaagttttgtggcaagatttctatcaaattgaatgttgtcttgtttcctatggtgggtgagacccaaggtgccagtgtttgaagtaatcattcagattggagtagcattttttcatgtgttactatattttccattcctttccagtcaacccagtaagataaatgctatttcaggggatatggtatctacaaaatttttcatttggatgtgtttgtatttgctaagtacaaatctacaccaatattgtcacttgtatattgtaccaacatatggcaggaaagcctggctggtcacaccaagtcttatttttcatcttgggatacgagttgccaacgatctgatatgacttgaaaaacaaacagacaaatctgcatcactaaaaaggcttatgtttctttaaaacatttcaaataaataattcatattaacgaaaaccgtccagccaagtcgaatactttgctgattgctatatttaattattgctaacaaattctgagcaggctgttttccagcatcctgtgcttttgtgagtgcggattccccactagtgggcgccatttgtcttcttattccttccgtgcagctcaccttaccgcaaattcatttataaatacaaaaatcagtgaaaggtgggggaagaagtgtgcaataaaaatcaaactcaactatagtgcagtccttagacaaggatttccttcaccctttcctgtttcctcattaaaacccagcaagaaagatgacttgagaatagcatttctatttaaatcctattggaaaataaattaataaacacacttgtaaaaatacggcagacttcaaaatgcagttaaaagataaaaaactctttgattagtaataaataaattataaaaatgtcacatttattttacatatactttacaaaaaaaaaaagagtacaatgaagaaataaaagaaaaacatatgaaaataaataagatctaataattgactgcattgcttttaatccaagaagtctatcatagtttttctttcctttttatatcagctggggaaaataaaattagtgcaatgttgcaaattgtaaatgcagtacggcaacctccacgccttagcagtacatgaacctctaacagatccatctggagtttactgctgttggtaacttctgttgcccggcagcgctgtgatcctacacatggatacccttcactgcctgtttgatactttccagtagagctttgcattccggggaatagtcccgttccagattgctgtacatatctgtgagtgtatttacatatgcttcaaaattctgctcactgataggtcccatctgtggaagctggatgtcagcaaggcttgaaatgagagcttggcttagacctgccagctctttcagcagactttcattgttctgttctatgagtttgttctcctcctctatcgtctttaagttgctctccatagatgtgatctgggtctgaagtttcatcatatctgcttcaattttaaggttggattcattcagttcctttatttcttcatccaaatgcctaatttcttcatcactctctattcccccagttgctttgagcttgatggtcatgagttcttcagaaaccttgccctttttgataacttgtgcattgagaggacatccagataagcttcggtgggtgacaaaaacattatttacatggcccagcccattgcagcctggcaagggacaatgtggtagctcttgtttgttcagtttccaggagagggaggctccattgagaggattctccttctgtctcttggcagccagaggacagccagaagctgtgcggtgtgatgtgtatttacctgatatgtgaccttggccatcacaccctatcacaggacatttcagttcagggtcttctttttcttccttggtaggggtcattttgacaccacctttccttgcacgagggcatccggacaagcttctgtgggaagcatagtttccagtcacgtgccccgagccatcgcagcctggggttggacacttaagctcctgagagttggcagccatgagggattttagagtcttatctgctaaaggacatccagaaacactgcgatgagatgcatagtttcctgtcacgtggccacttccatcacatcctggtgttggacaggtgattagttcctttttgagatctcttgcatgaagcttgggtttagggcttggtatagaggcctctccaggaaactttttttcctctaaattttctagagagctcactgggtctttctctttctcctcctctgtcttcccgtgagttttgctatagttgataggagtgtcccagccctcttggtcacaaagagcctgatagaatgctgcattgaccagaatgctgcttgttttgaatggggaagaggaaggagttggaatagaagtgttagaggaagttaggggtgcagacttgtccaggattcgattttttttcatgcttaagtccaatgtgccattttcatccacttctatttcggctcccttggcatgcagactctgtggcttgttggagaggatgtctgtggcttccctgcagcgggtggaaaggttcaggatggcagcagctgctgctatgtgggtgtcttcactacattgaccgtagctataagagctggcacggccagggctctgggtgtgggcgcctgcactaggcagtcgattaggaaatttcactggatttggaaaatgctttgattcaggaaatggtggtgtttttcgtccttgcactgtttgtatgagagggcgtttaccgaaaacttgggcatcaaaactggcataatcaaatggtacttttccaaacttctcttgttcttttgacactgtggctctgggagaggtgatggcttgtgacgggaaattgaattcaatttgcttcaccaaacttgtcctgtgggcctggtcaggacactgcccagtttggggagaatcaagctgatttttatcctgggacattgccaatttttcagctgcagcaattggacaaccagaaagactcctgtgggtgttgcggttgctgttcacatgaccccttcctgtgcatcccggcgtgggacacttgagcacattttcatgcatggcaagaatttccaggggaacccgcactttgtgggggcaccccgaaaggctgcggtggtgcgggtagagccctgtcacgtgtcccgtgccatcacatccagggatcgggcacttggtctccctcttttcaggccttggtgaatgtttattgttaaagatttgtcttccacccatgtcgataactttggtttgcctcctttcccctgctaggtgctccagcaggaacctatccagctctttgtaggtgttatggaaaacacaacctcgctcagcctgcagagcaattgcctgctccagcaaacttaaattccccttggccttttccaggtcactaccctcttccgtcattactgccaggctctcgctatcttcctcctcaacgtcagggaatgagggctgggcattgccatccaggggttctgcgagagcattctgcgggtctttcctttctgtttcagaatcacacctgttctcacaagggataaatttgtcaccttcagtttttatttcaggaacttccaataggtcttttttatgatctgttaaaacatactttgggactctaggtggtttggtttcttctgagaagttggagccactgtcccagccattttctgcactttcagagttactttcattgtcatcagaggagcagaagggtggctgagaatcatcaatcttgtctcttccatcatcagaatgaatcagaaagcactcgtctgcttcatcgctctctgcttttaaagactggatgccactgtcatttaaattttcacttacagtctgaacagatacatttttttcaaatttccccaagtgcattaaagacttgaccatgagctcttgataacaagagtatctgtcttccttcctactggagttttcttgtgcagttgaaagaagactttcatccataggttttatcatgatttcctctgcggtagagtgaccatgtgtttccaaggggccatcgtcctctgtcctgtcactgcggtcttcttggcagtctgcttttgggctgtagtgtcggggcttcattagcagggatttccttttgttgactggaacccccaaagcctgatcttcagctgttctcttctttgccatggagcaatcataggcaacactgagatcaggagttcgagaccagccggaccaacatggagaaacccgtctctactaaaaatacaaaattagcccggcatggtggctcatgcctgtaatcccagctactcgacaggctgaggcaagagaatcacttgaacccaggaggcggaggttgcagtgaaccgagatcgtgccattgcactccagcttgggcaacaagagcgaaactccatctgagctcctggattagtgaatccattggcacctcggttcctttagagcgagtacgcagcgttttatcttcagcctctgcatccatctataaacagatgtataaagtgatttcctagtacttgtacttgacgtcttttcttactggagcttacatcaggggcaataagcaggtctcttccacatcgccccagtgcacagatctggtaccttcttttaggctgaagaggaagtcctggaattgctctctttttctccaggtaacttgtatgtcaactcagtttgccctgctgtgtcagggggactaaataaatgactttgtcttatttagtgataaatcctgaaattcattctttcttgcagaaaatttctaccgtcctgccttctctaccctttgcagtatatcaaagtgctcagctttttaatcatagatttctgtgtttcttgtaggatttgaccagacattaaatagatgcttcttcaacttaagtcagcaactgtagttccttccctaaaagctactggatctgaactggagagtttccatcactcttttttgtttgtttccaaaacttatatttctctcctccctggtgggctgaacggaaacactaaagctgtttctttgaaaggtagttcccatgatatgac

SEQ ID NO: 18663 - RNA, 5046 nt, Homo sapiens
  source 1..5046: mol_type = other RNA
tgagtgtgtgtgtgtgagtgtgtgtgtatattttgtagcatttgaagttttgtggcaagatttctatcaaattgaatgttgtcttgtttcctatggtgggtgagacccaaggtgccagtgtttgaagtaatcattcagattggagtagcattttttcatgtgttactatattttccattcctttccagtcaacccagtaagataaatgctatttcaggggatatggtatctacaaaatttttcatttggatgtgtttgtatttgctaagtacaaatctacaccaatattgtcacttgtatattgtaccaacatatggcaggaaagcctggctggtcacaccaagtcttatttttcatcttgggatacgagttgccaacgatctgatatgacttgaaaaacaaacagacaaatctgcatcactaaaaaggcttatgtttctttaaaacatttcaaataaataattcatattaacgaaaaccgtccagccaagtcgaatactttgctgattgctatatttaattattgctaacaaattctgagcaggctgttttccagcatcctgtgcttttgtgagtgcggattccccactagtgggcgccatttgtcttcttattccttccgtgcagctcaccttaccgcaaattcatttataaatacaaaaatcagtgaaaggtgggggaagaagtgtgcaataaaaatcaaactcaactatagtgcagtccttagacaaggatttccttcaccctttcctgtttcctcattaaaacccagcaagaaagatgacttgagaatagcatttctatttaaatcctattggaaaataaattaataaacacacttgtaaaaatacggcagacttcaaaatgcagttaaaagataaaaaactctttgattagtaataaataaattataaaaatgtcacatttattttacatatactttacaaaaaaaaaaagagtacaatgaagaaataaaagaaaaacatatgaaaataaataagatctaataattgactgcattgcttttaatccaagaagtctatcatagtttttctttcctttttatatcagctggggaaaataaaattagtgcaatgttgcaaattgtaaatgcagtacggcaacctccacgccttagcagtacatgaacctctaacagatccatctggagtttactgctgttggtaacttctgttgcccggcagcgctgtgatcctacacatggatacccttcactgcctgtttgatactttccagtagagctttgcattccggggaatagtcccgttccagattgctgtacatatctgtgagtgtatttacatatgcttcaaaattctgctcactgataggtcccatctgtggaagctggatgtcagcaaggcttgaaatgagagcttggcttagacctgccagctctttcagcagactttcattgttctgttctatgagtttgttctcctcctctatcgtctttaagttgctctccatagatgtgatctgggtctgaagtttcatcatatctgcttcaattttaaggttggattcattcagttcctttatttcttcatccaaatgcctaatttcttcatcactctctattcccccagttgctttgagcttgatggtcatgagttcttcagaaaccttgccctttttgataacttgtgcattgagaggacatccagataagcttcggtgggtgacaaaaacattatttacatggcccagcccattgcagcctggcaagggacaatgtggtagctcttgtttgttcagtttccaggagagggaggctccattgagaggattctccttctgtctcttggcagccagaggacagccagaagctgtgcggtgtgatgtgtatttacctgatatgtgaccttggccatcacaccctatcacaggacatttcagttcagggtcttctttttcttccttggtaggggtcattttgacaccacctttccttgcacgagggcatccggacaagcttctgtgggaagcatagtttccagtcacgtgccccgagccatcgcagcctggggttggacacttaagctcctgagagttggcagccatgagggattttagagtcttatctgctaaaggacatccagaaacactgcgatgagatgcatagtttcctgtcacgtggccacttccatcacatcctggtgttggacaggtgattagttcctttttgagatctcttgcatgaagcttgggtttagggcttggtatagaggcctctccaggaaactttttttcctctaaattttctagagagctcactgggtctttctctttctcctcctctgtcttcccgtgagttttgctatagttgataggagtgtcccagccctcttggtcacaaagagcctgatagaatgctgcattgaccagaatgctgcttgttttgaatggggaagaggaaggagttggaatagaagtgttagaggaagttaggggtgcagacttgtccaggattcgattttttttcatgcttaagtccaatgtgccattttcatccacttctatttcggctcccttggcatgcagactctgtggcttgttggagaggatgtctgtggcttccctgcagcgggtggaaaggttcaggatggcagcagctgctgctatgtgggtgtcttcactacattgaccgtagctataagagctggcacggccagggctctgggtgtgggcgcctgcactaggcagtcgattaggaaatttcactggatttggaaaatgctttgattcaggaaatggtggtgtttttcgtccttgcactgtttgtatgagagggcgtttaccgaaaacttgggcatcaaaactggcataatcaaatggtacttttccaaacttctcttgttcttttgacactgtggctctgggagaggtgatggcttgtgacgggaaattgaattcaatttgcttcaccaaacttgtcctgtgggcctggtcaggacactgcccagtttggggagaatcaagctgatttttatcctgggacattgccaatttttcagctgcagcaattggacaaccagaaagactcctgtgggtgttgcggttgctgttcacatgaccccttcctgtgcatcccggcgtgggacacttgagcacattttcatgcatggcaagaatttccaggggaacccgcactttgtgggggcaccccgaaaggctgcggtggtgcgggtagagccctgtcacgtgtcccgtgccatcacatccagggatcgggcacttggtctccctcttttcaggccttggtgaatgtttattgttaaagatttgtcttccacccatgtcgataactttggtttgcctcctttcccctgctaggtgctccagcaggaacctatccagctctttgtaggtgttatggaaaacacaacctcgctcagcctgcagagcaattgcctgctccagcaaacttaaattccccttggccttttccaggtcactaccctcttccgtcattactgccaggctctcgctatcttcctcctcaacgtcagggaatgagggctgggcattgccatccaggggttctgcgagagcattctgcgggtctttcctttctgtttcagaatcacacctgttctcacaagggataaatttgtcaccttcagtttttatttcaggaacttccaataggtcttttttatgatctgttaaaacatactttgggactctaggtggtttggtttcttctgagaagttggagccactgtcccagccattttctgcactttcagagttactttcattgtcatcagaggagcagaagggtggctgagaatcatcaatcttgtctcttccatcatcagaatgaatcagaaagcactcgtctgcttcatcgctctctgcttttaaagactggatgccactgtcatttaaattttcacttacagtctgaacagatacatttttttcaaatttccccaagtgcattaaagacttgaccatgagctcttgataacaagagtatctgtcttccttcctactggagttttcttgtgcagttgaaagaagactttcatccataggttttatcatgatttcctctgcggtagagtgaccatgtgtttccaaggggccatcgtcctctgtcctgtcactgcggtcttcttggcagtctgcttttgggctgtagtgtcggggcttcattagcagggatttccttttgttgactggaacccccaaagcctgatcttcagctgttctcttctttgccatggagcaatcataggcaacactgagctcctggattagtgaatccattggcacctcggttcctttagagcgagtacgcagcgttttatcttcagcctctgcatccataaacctataaacagatgtataaagtgatttcctagtacttgtacttgacgtcttttcttactggagcttacatcaggggcaataagcaggtctcttccacatcgccccagtgcacagatctggtaccttcttttaggctgaagaggaagtcctggaattgctctctttttctccaggtaacttgtatgtcaactcagtttgccctgctgtgtcagggggactaaataaatgactttgtcttatttagtgataaatcctgaaattcattctttcttgcagaaaatttctaccgtcctgccttctctaccctttgcagtatatcaaagtgctcagctttttaatcatagatttctgtgtttcttgtaggatttgaccagacattaaatagatgcttcttcaacttaagtcagcaactgtagttcactagtaggcataacagtatttgtatttgtccttccagtcccttccctaaaagctactggatctgaactggagagtttccatcactccttagtcttgatatgagcacgcagacacataaaatggaattgtcacaatgcttcagggacactcacaaaattgggggctttttttgtttgtttccaaaacttatatttctctcctccctggtgggctgaacggaaacactaaagctgtttctttgaaaggtagttcccatgatatgac

SEQ ID NO: 18664 - RNA, 4957 nt, Homo sapiens
  source 1..4957: mol_type = other RNA
tgagtgtgtgtgtgtgagtgtgtgtgtatattttgtagcatttgaagttttgtggcaagatttctatcaaattgaatgttgtcttgtttcctatggtgggtgagacccaaggtgccagtgtttgaagtaatcattcagattggagtagcattttttcatgtgttactatattttccattcctttccagtcaacccagtaagataaatgctatttcaggggatatggtatctacaaaatttttcatttggatgtgtttgtatttgctaagtacaaatctacaccaatattgtcacttgtatattgtaccaacatatggcaggaaagcctggctggtcacaccaagtcttatttttcatcttgggatacgagttgccaacgatctgatatgacttgaaaaacaaacagacaaatctgcatcactaaaaaggcttatgtttctttaaaacatttcaaataaataattcatattaacgaaaaccgtccagccaagtcgaatactttgctgattgctatatttaattattgctaacaaattctgagcaggctgttttccagcatcctgtgcttttgtgagtgcggattccccactagtgggcgccatttgtcttcttattccttccgtgcagctcaccttaccgcaaattcatttataaatacaaaaatcagtgaaaggtgggggaagaagtgtgcaataaaaatcaaactcaactatagtgcagtccttagacaaggatttccttcaccctttcctgtttcctcattaaaacccagcaagaaagatgacttgagaatagcatttctatttaaatcctattggaaaataaattaataaacacacttgtaaaaatacggcagacttcaaaatgcagttaaaagataaaaaactctttgattagtaataaataaattataaaaatgtcacatttattttacatatactttacaaaaaaaaaaagagtacaatgaagaaataaaagaaaaacatatgaaaataaataagatctaataattgactgcattgcttttaatccaagaagtctatcatagtttttctttcctttttatatcagctggggaaaataaaattagtgcaatgttgcaaattgtaaatgcagtacggcaacctccacgccttagcagtacatgaacctctaacagatccatctggagtttactgctgttggtaacttctgttgcccggcagcgctgtgatcctacacatggatacccttcactgcctgtttgatactttccagtagagctttgcattccggggaatagtcccgttccagattgctgtacatatctgtgagtgtatttacatatgcttcaaaattctgctcactgataggtcccatctgtggaagctggatgtcagcaaggcttgaaatgagagcttggcttagacctgccagctctttcagcagactttcattgttctgttctatgagtttgttctcctcctctatcgtctttaagttgctctccatagatgtgatctgggtctgaagtttcatcatatctgcttcaattttaaggttggattcattcagttcctttatttcttcatccaaatgcctaatttcttcatcactctctattcccccagttgctttgagcttgatggtcatgagttcttcagaaaccttgccctttttgataacttgtgcattgagaggacatccagataagcttcggtgggtgacaaaaacattatttacatggcccagcccattgcagcctggcaagggacaatgtggtagctcttgtttgttcagtttccaggagagggaggctccattgagaggattctccttctgtctcttggcagccagaggacagccagaagctgtgcggtgtgatgtgtatttacctgatatgtgaccttggccatcacaccctatcacaggacatttcagttcagggtcttctttttcttccttggtaggggtcattttgacaccacctttccttgcacgagggcatccggacaagcttctgtgggaagcatagtttccagtcacgtgccccgagccatcgcagcctggggttggacacttaagctcctgagagttggcagccatgagggattttagagtcttatctgctaaaggacatccagaaacactgcgatgagatgcatagtttcctgtcacgtggccacttccatcacatcctggtgttggacaggtgattagttcctttttgagatctcttgcatgaagcttgggtttagggcttggtatagaggcctctccaggaaactttttttcctctaaattttctagagagctcactgggtctttctctttctcctcctctgtcttcccgtgagttttgctatagttgataggagtgtcccagccctcttggtcacaaagagcctgatagaatgctgcattgaccagaatgctgcttgttttgaatggggaagaggaaggagttggaatagaagtgttagaggaagttaggggtgcagacttgtccaggattcgattttttttcatgcttaagtccaatgtgccattttcatccacttctatttcggctcccttggcatgcagactctgtggcttgttggagaggatgtctgtggcttccctgcagcgggtggaaaggttcaggatggcagcagctgctgctatgtgggtgtcttcactacattgaccgtagctataagagctggcacggccagggctctgggtgtgggcgcctgcactaggcagtcgattaggaaatttcactggatttggaaaatgctttgattcaggaaatggtggtgtttttcgtccttgcactgtttgtatgagagggcgtttaccgaaaacttgggcatcaaaactggcataatcaaatggtacttttccaaacttctcttgttcttttgacactgtggctctgggagaggtgatggcttgtgacgggaaattgaattcaatttgcttcaccaaacttgtcctgtgggcctggtcaggacactgcccagtttggggagaatcaagctgatttttatcctgggacattgccaatttttcagctgcagcaattggacaaccagaaagactcctgtgggtgttgcggttgctgttcacatgaccccttcctgtgcatcccggcgtgggacacttgagcacattttcatgcatggcaagaatttccaggggaacccgcactttgtgggggcaccccgaaaggctgcggtggtgcgggtagagccctgtcacgtgtcccgtgccatcacatccagggatcgggcacttggtctccctcttttcaggccttggtgaatgtttattgttaaagatttgtcttccacccatgtcgataactttggtttgcctcctttcccctgctaggtgctccagcaggaacctatccagctctttgtaggtgttatggaaaacacaacctcgctcagcctgcagagcaattgcctgctccagcaaacttaaattccccttggccttttccaggtcactaccctcttccgtcattactgccaggctctcgctatcttcctcctcaacgtcagggaatgagggctgggcattgccatccaggggttctgcgagagcattctgcgggtctttcctttctgtttcagaatcacacctgttctcacaagggataaatttgtcaccttcagtttttatttcaggaacttccaataggtcttttttatgatctgttaaaacatactttgggactctaggtggtttggtttcttctgagaagttggagccactgtcccagccattttctgcactttcagagttactttcattgtcatcagaggagcagaagggtggctgagaatcatcaatcttgtctcttccatcatcagaatgaatcagaaagcactcgtctgcttcatcgctctctgcttttaaagactggatgccactgtcatttaaattttcacttacagtctgaacagatacatttttttcaaatttccccaagtgcattaaagacttgaccatgagctcttgataacaagagtatctgtcttccttcctactggagttttcttgtgcagttgaaagaagactttcatccataggttttatcatgatttcctctgcggtagagtgaccatgtgtttccaaggggccatcgtcctctgtcctgtcactgcggtcttcttggcagtctgcttttgggctgtagtgtcggggcttcattagcagggatttccttttgttgactggaacccccaaagcctgatcttcagctgttctcttctttgccatggagcaatcataggcaacactgagctcctggattagtgaatccattggcacctcggttcctttagagcgagtacgcagcgttttatcttcagcctctgcatccataaacctataaacagatgtataaagtgatttcctagtacttgtacttgacgtcttttcttactggagcttacatcaggggcaataagcaggtctcttccacatcgccccagtgcacagatctggtaccttcttttaggctgaagaggaagtcctggaattgctctctttttctccaggtaacttgtatgtcaactcagtttgccctgctgtgtcagggggactaaataaatgactttgtcttatttagtgataaatcctgaaattcattctttcttgcagaaaatttctaccgtcctgccttctctaccctttgcagtatatcaaagtgctcagctttttaatcatagatttctgtgtttcttgtaggatttgaccagacattaaatagatgcttcttcaacttaagtcagcaactgtagttccttccctaaaagctactggatctgaactggagagtttccatcactccggtgcctcctagcctttgttctgcctctcacgctgacatcagggaagcagtgatgtagaataaagcaggggtgggctaggttagtccagtgtttgtgtcgttgtgtggtgtgcagggacactctgtgat

SEQ ID NO: 18665 - RNA, 4961 nt, Homo sapiens
  source 1..4961: mol_type = other RNA
tgagtgtgtgtgtgtgagtgtgtgtgtatattttgtagcatttgaagttttgtggcaagatttctatcaaattgaatgttgtcttgtttcctatggtgggtgagacccaaggtgccagtgtttgaagtaatcattcagattggagtagcattttttcatgtgttactatattttccattcctttccagtcaacccagtaagataaatgctatttcaggggatatggtatctacaaaatttttcatttggatgtgtttgtatttgctaagtacaaatctacaccaatattgtcacttgtatattgtaccaacatatggcaggaaagcctggctggtcacaccaagtcttatttttcatcttgggatacgagttgccaacgatctgatatgacttgaaaaacaaacagacaaatctgcatcactaaaaaggcttatgtttctttaaaacatttcaaataaataattcatattaacgaaaaccgtccagccaagtcgaatactttgctgattgctatatttaattattgctaacaaattctgagcaggctgttttccagcatcctgtgcttttgtgagtgcggattccccactagtgggcgccatttgtcttcttattccttccgtgcagctcaccttaccgcaaattcatttataaatacaaaaatcagtgaaaggtgggggaagaagtgtgcaataaaaatcaaactcaactatagtgcagtccttagacaaggatttccttcaccctttcctgtttcctcattaaaacccagcaagaaagatgacttgagaatagcatttctatttaaatcctattggaaaataaattaataaacacacttgtaaaaatacggcagacttcaaaatgcagttaaaagataaaaaactctttgattagtaataaataaattataaaaatgtcacatttattttacatatactttacaaaaaaaaaaagagtacaatgaagaaataaaagaaaaacatatgaaaataaataagatctaataattgactgcattgcttttaatccaagaagtctatcatagtttttctttcctttttatatcagctggggaaaataaaattagtgcaatgttgcaaattgtaaatgcagtacggcaacctccacgccttagcagtacatgaacctctaacagatccatctggagtttactgctgttggtaacttctgttgcccggcagcgctgtgatcctacacatggatacccttcactgcctgtttgatactttccagtagagctttgcattccggggaatagtcccgttccagattgctgtacatatctgtgagtgtatttacatatgcttcaaaattctgctcactgataggtcccatctgtggaagctggatgtcagcaaggcttgaaatgagagcttggcttagacctgccagctctttcagcagactttcattgttctgttctatgagtttgttctcctcctctatcgtctttaagttgctctccatagatgtgatctgggtctgaagtttcatcatatctgcttcaattttaaggttggattcattcagttcctttatttcttcatccaaatgcctaatttcttcatcactctctattcccccagttgctttgagcttgatggtcatgagttcttcagaaaccttgccctttttgataacttgtgcattgagaggacatccagataagcttcggtgggtgacaaaaacattatttacatggcccagcccattgcagcctggcaagggacaatgtggtagctcttgtttgttcagtttccaggagagggaggctccattgagaggattctccttctgtctcttggcagccagaggacagccagaagctgtgcggtgtgatgtgtatttacctgatatgtgaccttggccatcacaccctatcacaggacatttcagttcagggtcttctttttcttccttggtaggggtcattttgacaccacctttccttgcacgagggcatccggacaagcttctgtgggaagcatagtttccagtcacgtgccccgagccatcgcagcctggggttggacacttaagctcctgagagttggcagccatgagggattttagagtcttatctgctaaaggacatccagaaacactgcgatgagatgcatagtttcctgtcacgtggccacttccatcacatcctggtgttggacaggtgattagttcctttttgagatctcttgcatgaagcttgggtttagggcttggtatagaggcctctccaggaaactttttttcctctaaattttctagagagctcactgggtctttctctttctcctcctctgtcttcccgtgagttttgctatagttgataggagtgtcccagccctcttggtcacaaagagcctgatagaatgctgcattgaccagaatgctgcttgttttgaatggggaagaggaaggagttggaatagaagtgttagaggaagttaggggtgcagacttgtccaggattcgattttttttcatgcttaagtccaatgtgccattttcatccacttctatttcggctcccttggcatgcagactctgtggcttgttggagaggatgtctgtggcttccctgcagcgggtggaaaggttcaggatggcagcagctgctgctatgtgggtgtcttcactacattgaccgtagctataagagctggcacggccagggctctgggtgtgggcgcctgcactaggcagtcgattaggaaatttcactggatttggaaaatgctttgattcaggaaatggtggtgtttttcgtccttgcactgtttgtatgagagggcgtttaccgaaaacttgggcatcaaaactggcataatcaaatggtacttttccaaacttctcttgttcttttgacactgtggctctgggagaggtgatggcttgtgacgggaaattgaattcaatttgcttcaccaaacttgtcctgtgggcctggtcaggacactgcccagtttggggagaatcaagctgatttttatcctgggacattgccaatttttcagctgcagcaattggacaaccagaaagactcctgtgggtgttgcggttgctgttcacatgaccccttcctgtgcatcccggcgtgggacacttgagcacattttcatgcatggcaagaatttccaggggaacccgcactttgtgggggcaccccgaaaggctgcggtggtgcgggtagagccctgtcacgtgtcccgtgccatcacatccagggatcgggcacttggtctccctcttttcaggccttggtgaatgtttattgttaaagatttgtcttccacccatgtcgataactttggtttgcctcctttcccctgctaggtgctccagcaggaacctatccagctctttgtaggtgttatggaaaacacaacctcgctcagcctgcagagcaattgcctgctccagcaaacttaaattccccttggccttttccaggtcactaccctcttccgtcattactgccaggctctcgctatcttcctcctcaacgtcagggaatgagggctgggcattgccatccaggggttctgcgagagcattctgcgggtctttcctttctgtttcagaatcacacctgttctcacaagggataaatttgtcaccttcagtttttatttcaggaacttccaataggtcttttttatgatctgttaaaacatactttgggactctaggtggtttggtttcttctgagaagttggagccactgtcccagccattttctgcactttcagagttactttcattgtcatcagaggagcagaagggtggctgagaatcatcaatcttgtctcttccatcatcagaatgaatcagaaagcactcgtctgcttcatcgctctctgcttttaaagactggatgccactgtcatttaaattttcacttacagtctgaacagatacatttttttcaaatttccccaagtgcattaaagacttgaccatgagctcttgataacaagagtatctgtcttccttcctactggagttttcttgtgcagttgaaagaagactttcatccataggttttatcatgatttcctctgcggtagagtgaccatgtgtttccaaggggccatcgtcctctgtcctgtcactgcggtcttcttggcagtctgcttttgggctgtagtgtcggggcttcattagcagggatttccttttgttgactggaacccccaaagcctgatcttcagctgttctcttctttgccatggagcaatcataggcaacactgagctcctggattagtgaatccattggcacctcggttcctttagagcgagtacgcagcgttttatcttcagcctctgcatccataaacctataaacagatgtataaagtgatttcctagtacttgtacttgacgtcttttcttactggagcttacatcaggggcaataagcaggtctcttccacatcgccccagtgcacagatctggtaccttcttttaggctgaagaggaagtcctggaattgctctctttttctccaggtaacttgtatgtcaactcagtttgccctgctgtgtcagggggactaaataaatgactttgtcttatttagtgataaatcctgaaattcattctttcttgcagaaaatttctaccgtcctgccttctctaccctttgcagtatatcaaagtgctcagctttttaatcatagatttctgtgtttcttgtaggatttgaccagacattaaatagatgcttcttcaacttaagtcagcaactgtagttccttccctaaaagctactggatctgaactggagagtttccatcactccttagtcttgatatgagcacgcagacacataaaatggaattgtcacaatgcttcagggacactcacaaaattgggggctcggtgcctcctagcctttgttctgcctctcacgctgacatcagggaagcagtgat

SEQ ID NO: 18666 - RNA, 5240 nt, Homo sapiens
  source 1..5240: mol_type = other RNA
tgagtgtgtgtgtgtgagtgtgtgtgtatattttgtagcatttgaagttttgtggcaagatttctatcaaattgaatgttgtcttgtttcctatggtgggtgagacccaaggtgccagtgtttgaagtaatcattcagattggagtagcattttttcatgtgttactatattttccattcctttccagtcaacccagtaagataaatgctatttcaggggatatggtatctacaaaatttttcatttggatgtgtttgtatttgctaagtacaaatctacaccaatattgtcacttgtatattgtaccaacatatggcaggaaagcctggctggtcacaccaagtcttatttttcatcttgggatacgagttgccaacgatctgatatgacttgaaaaacaaacagacaaatctgcatcactaaaaaggcttatgtttctttaaaacatttcaaataaataattcatattaacgaaaaccgtccagccaagtcgaatactttgctgattgctatatttaattattgctaacaaattctgagcaggctgttttccagcatcctgtgcttttgtgagtgcggattccccactagtgggcgccatttgtcttcttattccttccgtgcagctcaccttaccgcaaattcatttataaatacaaaaatcagtgaaaggtgggggaagaagtgtgcaataaaaatcaaactcaactatagtgcagtccttagacaaggatttccttcaccctttcctgtttcctcattaaaacccagcaagaaagatgacttgagaatagcatttctatttaaatcctattggaaaataaattaataaacacacttgtaaaaatacggcagacttcaaaatgcagttaaaagataaaaaactctttgattagtaataaataaattataaaaatgtcacatttattttacatatactttacaaaaaaaaaaagagtacaatgaagaaataaaagaaaaacatatgaaaataaataagatctaataattgactgcattgcttttaatccaagaagtctatcatagtttttctttcctttttatatcagctggggaaaataaaattagtgcaatgttgcaaattgtaaatgcagtacggcaacctccacgccttagcagtacatgaacctctaacagatccatctggagtttactgctgttggtaacttctgttgcccggcagcgctgtgatcctacacatggatacccttcactgcctgtttgatactttccagtagagctttgcattccggggaatagtcccgttccagattgctgtacatatctgtgagtgtatttacatatgcttcaaaattctgctcactgataggtcccatctgtggaagctggatgtcagcaaggcttgaaatgagagcttggcttagacctgccagctctttcagcagactttcattgttctgttctatgagtttgttctcctcctctatcgtctttaagttgctctccatagatgtgatctgggtctgaagtttcatcatatctgcttcaattttaaggttggattcattcagttcctttatttcttcatccaaatgcctaatttcttcatcactctctattcccccagttgctttgagcttgatggtcatgagttcttcagaaaccttgccctttttgataacttgtgcattgagaggacatccagataagcttcggtgggtgacaaaaacattatttacatggcccagcccattgcagcctggcaagggacaatgtggtagctcttgtttgttcagtttccaggagagggaggctccattgagaggattctccttctgtctcttggcagccagaggacagccagaagctgtgcggtgtgatgtgtatttacctgatatgtgaccttggccatcacaccctatcacaggacatttcagttcagggtcttctttttcttccttggtaggggtcattttgacaccacctttccttgcacgagggcatccggacaagcttctgtgggaagcatagtttccagtcacgtgccccgagccatcgcagcctggggttggacacttaagctcctgagagttggcagccatgagggattttagagtcttatctgctaaaggacatccagaaacactgcgatgagatgcatagtttcctgtcacgtggccacttccatcacatcctggtgttggacaggtgattagttcctttttgagatctcttgcatgaagcttgggtttagggcttggtatagaggcctctccaggaaactttttttcctctaaattttctagagagctcactgggtctttctctttctcctcctctgtcttcccgtgagttttgctatagttgataggagtgtcccagccctcttggtcacaaagagcctgatagaatgctgcattgaccagaatgctgcttgttttgaatggggaagaggaaggagttggaatagaagtgttagaggaagttaggggtgcagacttgtccaggattcgattttttttcatgcttaagtccaatgtgccattttcatccacttctatttcggctcccttggcatgcagactctgtggcttgttggagaggatgtctgtggcttccctgcagcgggtggaaaggttcaggatggcagcagctgctgctatgtgggtgtcttcactacattgaccgtagctataagagctggcacggccagggctctgggtgtgggcgcctgcactaggcagtcgattaggaaatttcactggatttggaaaatgctttgattcaggaaatggtggtgtttttcgtccttgcactgtttgtatgagagggcgtttaccgaaaacttgggcatcaaaactggcataatcaaatggtacttttccaaacttctcttgttcttttgacactgtggctctgggagaggtgatggcttgtgacgggaaattgaattcaatttgcttcaccaaacttgtcctgtgggcctggtcaggacactgcccagtttggggagaatcaagctgatttttatcctgggacattgccaatttttcagctgcagcaattggacaaccagaaagactcctgtgggtgttgcggttgctgttcacatgaccccttcctgtgcatcccggcgtgggacacttgagcacattttcatgcatggcaagaatttccaggggaacccgcactttgtgggggcaccccgaaaggctgcggtggtgcgggtagagccctgtcacgtgtcccgtgccatcacatccagggatcgggcacttggtctccctcttttcaggccttggtgaatgtttattgttaaagatttgtcttccacccatgtcgataactttggtttgcctcctttcccctgctaggtgctccagcaggaacctatccagctctttgtaggtgttatggaaaacacaacctcgctcagcctgcagagcaattgcctgctccagcaaacttaaattccccttggccttttccaggtcactaccctcttccgtcattactgccaggctctcgctatcttcctcctcaacgtcagggaatgagggctgggcattgccatccaggggttctgcgagagcattctgcgggtctttcctttctgtttcagaatcacacctgttctcacaagggataaatttgtcaccttcagtttttatttcaggaacttccaataggtcttttttatgatctgttaaaacatactttgggactctaggtggtttggtttcttctgagaagttggagccactgtcccagccattttctgcactttcagagttactttcattgtcatcagaggagcagaagggtggctgagaatcatcaatcttgtctcttccatcatcagaatgaatcagaaagcactcgtctgcttcatcgctctctgcttttaaagactggatgccactgtcatttaaattttcacttacagtctgaacagatacatttttttcaaatttccccaagtgcattaaagacttgaccatgagctcttgataacaagagtatctgtcttccttcctactggagttttcttgtgcagttgaaagaagactttcatccataggttttatcatgatttcctctgcggtagagtgaccatgtgtttccaaggggccatcgtcctctgtcctgtcactgcggtcttcttggcagtctgcttttgggctgtagtgtcggggcttcattagcagggatttccttttgttgactggaacccccaaagcctgatcttcagctgttctcttctttgccatggagcaatcataggcaacactgagctcctggattagtgaatccattggcacctcggttcctttagagcgagtacgcagcgttttatcttcagcctctgcatccataaacctataaacagatgtataaagtgatttcctagtacttgtacttgacgtcttttcttactggagcttacatcaggggcaataagcaggtctcttccacatcgccccagtgcacagatctggtaccttcttttaggctgaagaggaagtcctggaattgctctctttttctccaggtaacttgtatgtcaactcagtttgccctgctgtgtcagggggactaaataaatgactttgtcttatttagtgataaatcctgaaattcattctttcttgcagaaaatttctaccgtcctgccttctctaccctttgcagtatatcaaagtgctcagctttttaatcatagatttctgtgtttcttgtaggatttgaccagacattaaatagatgcttcttcaacttaagtcagcaactgtagttccttccctaaaagctactggatctgaactggagagtttccatcactccttagtcttgatatgagcacgcagacacataaaatggaattgtcacaatgcttcagggacactcacaaaattgggggctctttacctggcgaacgtctacaggtgtgtcgaaagttatcttttcctggatgtgttccaaaatgctcttatgctatttctcttaggatttctccacgctgccccattcagaaattttattattttcttccacaactctgccaggcactggtttttgcgtgggatgatgccagcttctctcttcatgtggccttattaaaagccatggtttccgagatgtaaaacacccacagttacctcaattatttttctctccttacctctagtattcccctgaggtcacattcagttaaaaacatcctgcccttctccctacaaaaaggttccatagaatc

SEQ ID NO: 18667 - RNA, 5005 nt, Homo sapiens
  source 1..5005: mol_type = other RNA
tgagtgtgtgtgtgtgagtgtgtgtgtatattttgtagcatttgaagttttgtggcaagatttctatcaaattgaatgttgtcttgtttcctatggtgggtgagacccaaggtgccagtgtttgaagtaatcattcagattggagtagcattttttcatgtgttactatattttccattcctttccagtcaacccagtaagataaatgctatttcaggggatatggtatctacaaaatttttcatttggatgtgtttgtatttgctaagtacaaatctacaccaatattgtcacttgtatattgtaccaacatatggcaggaaagcctggctggtcacaccaagtcttatttttcatcttgggatacgagttgccaacgatctgatatgacttgaaaaacaaacagacaaatctgcatcactaaaaaggcttatgtttctttaaaacatttcaaataaataattcatattaacgaaaaccgtccagccaagtcgaatactttgctgattgctatatttaattattgctaacaaattctgagcaggctgttttccagcatcctgtgcttttgtgagtgcggattccccactagtgggcgccatttgtcttcttattccttccgtgcagctcaccttaccgcaaattcatttataaatacaaaaatcagtgaaaggtgggggaagaagtgtgcaataaaaatcaaactcaactatagtgcagtccttagacaaggatttccttcaccctttcctgtttcctcattaaaacccagcaagaaagatgacttgagaatagcatttctatttaaatcctattggaaaataaattaataaacacacttgtaaaaatacggcagacttcaaaatgcagttaaaagataaaaaactctttgattagtaataaataaattataaaaatgtcacatttattttacatatactttacaaaaaaaaaaagagtacaatgaagaaataaaagaaaaacatatgaaaataaataagatctaataattgactgcattgcttttaatccaagaagtctatcatagtttttctttcctttttatatcagctggggaaaataaaattagtgcaatgttgcaaattgtaaatgcagtacggcaacctccacgccttagcagtacatgaacctctaacagatccatctggagtttactgctgttggtaacttctgttgcccggcagcgctgtgatcctacacatggatacccttcactgcctgtttgatactttccagtagagctttgcattccggggaatagtcccgttccagattgctgtacatatctgtgagtgtatttacatatgcttcaaaattctgctcactgataggtcccatctgtggaagctggatgtcagcaaggcttgaaatgagagcttggcttagacctgccagctctttcagcagactttcattgttctgttctatgagtttgttctcctcctctatcgtctttaagttgctctccatagatgtgatctgggtctgaagtttcatcatatctgcttcaattttaaggttggattcattcagttcctttatttcttcatccaaatgcctaatttcttcatcactctctattcccccagttgctttgagcttgatggtcatgagttcttcagaaaccttgccctttttgataacttgtgcattgagaggacatccagataagcttcggtgggtgacaaaaacattatttacatggcccagcccattgcagcctggcaagggacaatgtggtagctcttgtttgttcagtttccaggagagggaggctccattgagaggattctccttctgtctcttggcagccagaggacagccagaagctgtgcggtgtgatgtgtatttacctgatatgtgaccttggccatcacaccctatcacaggacatttcagttcagggtcttctttttcttccttggtaggggtcattttgacaccacctttccttgcacgagggcatccggacaagcttctgtgggaagcatagtttccagtcacgtgccccgagccatcgcagcctggggttggacacttaagctcctgagagttggcagccatgagggattttagagtcttatctgctaaaggacatccagaaacactgcgatgagatgcatagtttcctgtcacgtggccacttccatcacatcctggtgttggacaggtgattagttcctttttgagatctcttgcatgaagcttgggtttagggcttggtatagaggcctctccaggaaactttttttcctctaaattttctagagagctcactgggtctttctctttctcctcctctgtcttcccgtgagttttgctatagttgataggagtgtcccagccctcttggtcacaaagagcctgatagaatgctgcattgaccagaatgctgcttgttttgaatggggaagaggaaggagttggaatagaagtgttagaggaagttaggggtgcagacttgtccaggattcgattttttttcatgcttaagtccaatgtgccattttcatccacttctatttcggctcccttggcatgcagactctgtggcttgttggagaggatgtctgtggcttccctgcagcgggtggaaaggttcaggatggcagcagctgctgctatgtgggtgtcttcactacattgaccgtagctataagagctggcacggccagggctctgggtgtgggcgcctgcactaggcagtcgattaggaaatttcactggatttggaaaatgctttgattcaggaaatggtggtgtttttcgtccttgcactgtttgtatgagagggcgtttaccgaaaacttgggcatcaaaactggcataatcaaatggtacttttccaaacttctcttgttcttttgacactgtggctctgggagaggtgatggcttgtgacgggaaattgaattcaatttgcttcaccaaacttgtcctgtgggcctggtcaggacactgcccagtttggggagaatcaagctgatttttatcctgggacattgccaatttttcagctgcagcaattggacaaccagaaagactcctgtgggtgttgcggttgctgttcacatgaccccttcctgtgcatcccggcgtgggacacttgagcacattttcatgcatggcaagaatttccaggggaacccgcactttgtgggggcaccccgaaaggctgcggtggtgcgggtagagccctgtcacgtgtcccgtgccatcacatccagggatcgggcacttggtctccctcttttcaggccttggtgaatgtttattgttaaagatttgtcttccacccatgtcgataactttggtttgcctcctttcccctgctaggtgctccagcaggaacctatccagctctttgtaggtgttatggaaaacacaacctcgctcagcctgcagagcaattgcctgctccagcaaacttaaattccccttggccttttccaggtcactaccctcttccgtcattactgccaggctctcgctatcttcctcctcaacgtcagggaatgagggctgggcattgccatccaggggttctgcgagagcattctgcgggtctttcctttctgtttcagaatcacacctgttctcacaagggataaatttgtcaccttcagtttttatttcaggaacttccaataggtcttttttatgatctgttaaaacatactttgggactctaggtggtttggtttcttctgagaagttggagccactgtcccagccattttctgcactttcagagttactttcattgtcatcagaggagcagaagggtggctgagaatcatcaatcttgtctcttccatcatcagaatgaatcagaaagcactcgtctgcttcatcgctctctgcttttaaagactggatgccactgtcatttaaattttcacttacagtctgaacagatacatttttttcaaatttccccaagtgcattaaagacttgaccatgagctcttgataacaagagtatctgtcttccttcctactggagttttcttgtgcagttgaaagaagactttcatccataggttttatcatgatttcctctgcggtagagtgaccatgtgtttccaaggggccatcgtcctctgtcctgtcactgcggtcttcttggcagtctgcttttgggctgtagtgtcggggcttcattagcagggatttccttttgttgactggaacccccaaagcctgatcttcagctgttctcttctttgccatggagcaatcataggcaacactgagctcctggattagtgaatccattggcacctcggttcctttagagcgagtacgcagcgttttatcttcagcctctgcatccataaacctataaacagatgtataaagtgatttcctagtacttgtacttgacgtcttttcttactggagcttacatcaggggcaataagcaggtctcttccacatcgccccagtgcacagatctggtaccttcttttaggctgaagaggaagtcctggaattgctctctttttctccaggtaacttgtatgtcaactcagtttgccctgctgtgtcagggggactaaataaatgactttgtcttatttagtgataaatcctgaaattcattctttcttgcagaaaatttctaccgtcctgccttctctaccctttgcagtatatcaaagtgctcagctttttaatcatagatttctgtgtttcttgtaggatttgaccagacattaaatagatgcttcttcaacttaagtcagcaactgtagttccttccctaaaagctactggatctgaactggagagtttccatcactccttagtcttgatatgagcacgcagacacataaaatggaattgtcacaatgcttcagggacactcacaaaattgggggctttttttgtttgtttccaaaacttatatttctctcctccctggtgggctgaacggaaacactaaagctgtttctttgaaaggtagttcccatgatatgac

SEQ ID NO: 18668 - RNA, 5150 nt, Homo sapiens
  source 1..5150: mol_type = other RNA
tgagtgtgtgtgtgtgagtgtgtgtgtatattttgtagcatttgaagttttgtggcaagatttctatcaaattgaatgttgtcttgtttcctatggtgggtgagacccaaggtgccagtgtttgaagtaatcattcagattggagtagcattttttcatgtgttactatattttccattcctttccagtcaacccagtaagataaatgctatttcaggggatatggtatctacaaaatttttcatttggatgtgtttgtatttgctaagtacaaatctacaccaatattgtcacttgtatattgtaccaacatatggcaggaaagcctggctggtcacaccaagtcttatttttcatcttgggatacgagttgccaacgatctgatatgacttgaaaaacaaacagacaaatctgcatcactaaaaaggcttatgtttctttaaaacatttcaaataaataattcatattaacgaaaaccgtccagccaagtcgaatactttgctgattgctatatttaattattgctaacaaattctgagcaggctgttttccagcatcctgtgcttttgtgagtgcggattccccactagtgggcgccatttgtcttcttattccttccgtgcagctcaccttaccgcaaattcatttataaatacaaaaatcagtgaaaggtgggggaagaagtgtgcaataaaaatcaaactcaactatagtgcagtccttagacaaggatttccttcaccctttcctgtttcctcattaaaacccagcaagaaagatgacttgagaatagcatttctatttaaatcctattggaaaataaattaataaacacacttgtaaaaatacggcagacttcaaaatgcagttaaaagataaaaaactctttgattagtaataaataaattataaaaatgtcacatttattttacatatactttacaaaaaaaaaaagagtacaatgaagaaataaaagaaaaacatatgaaaataaataagatctaataattgactgcattgcttttaatccaagaagtctatcatagtttttctttcctttttatatcagctggggaaaataaaattagtgcaatgttgcaaattgtaaatgcagtacggcaacctccacgccttagcagtacatgaacctctaacagatccatctggagtttactgctgttggtaacttctgttgcccggcagcgctgtgatcctacacatggatacccttcactgcctgtttgatactttccagtagagctttgcattccggggaatagtcccgttccagattgctgtacatatctgtgagtgtatttacatatgcttcaaaattctgctcactgataggtcccatctgtggaagctggatgtcagcaaggcttgaaatgagagcttggcttagacctgccagctctttcagcagactttcattgttctgttctatgagtttgttctcctcctctatcgtctttaagttgctctccatagatgtgatctgggtctgaagtttcatcatatctgcttcaattttaaggttggattcattcagttcctttatttcttcatccaaatgcctaatttcttcatcactctctattcccccagttgctttgagcttgatggtcatgagttcttcagaaaccttgccctttttgataacttgtgcattgagaggacatccagataagcttcggtgggtgacaaaaacattatttacatggcccagcccattgcagcctggcaagggacaatgtggtagctcttgtttgttcagtttccaggagagggaggctccattgagaggattctccttctgtctcttggcagccagaggacagccagaagctgtgcggtgtgatgtgtatttacctgatatgtgaccttggccatcacaccctatcacaggacatttcagttcagggtcttctttttcttccttggtaggggtcattttgacaccacctttccttgcacgagggcatccggacaagcttctgtgggaagcatagtttccagtcacgtgccccgagccatcgcagcctggggttggacacttaagctcctgagagttggcagccatgagggattttagagtcttatctgctaaaggacatccagaaacactgcgatgagatgcatagtttcctgtcacgtggccacttccatcacatcctggtgttggacaggtgattagttcctttttgagatctcttgcatgaagcttgggtttagggcttggtatagaggcctctccaggaaactttttttcctctaaattttctagagagctcactgggtctttctctttctcctcctctgtcttcccgtgagttttgctatagttgataggagtgtcccagccctcttggtcacaaagagcctgatagaatgctgcattgaccagaatgctgcttgttttgaatggggaagaggaaggagttggaatagaagtgttagaggaagttaggggtgcagacttgtccaggattcgattttttttcatgcttaagtccaatgtgccattttcatccacttctatttcggctcccttggcatgcagactctgtggcttgttggagaggatgtctgtggcttccctgcagcgggtggaaaggttcaggatggcagcagctgctgctatgtgggtgtcttcactacattgaccgtagctataagagctggcacggccagggctctgggtgtgggcgcctgcactaggcagtcgattaggaaatttcactggatttggaaaatgctttgattcaggaaatggtggtgtttttcgtccttgcactgtttgtatgagagggcgtttaccgaaaacttgggcatcaaaactggcataatcaaatggtacttttccaaacttctcttgttcttttgacactgtggctctgggagaggtgatggcttgtgacgggaaattgaattcaatttgcttcaccaaacttgtcctgtgggcctggtcaggacactgcccagtttggggagaatcaagctgatttttatcctgggacattgccaatttttcagctgcagcaattggacaaccagaaagactcctgtgggtgttgcggttgctgttcacatgaccccttcctgtgcatcccggcgtgggacacttgagcacattttcatgcatggcaagaatttccaggggaacccgcactttgtgggggcaccccgaaaggctgcggtggtgcgggtagagccctgtcacgtgtcccgtgccatcacatccagggatcgggcacttggtctccctcttttcaggccttggtgaatgtttattgttaaagatttgtcttccacccatgtcgataactttggtttgcctcctttcccctgctaggtgctccagcaggaacctatccagctctttgtaggtgttatggaaaacacaacctcgctcagcctgcagagcaattgcctgctccagcaaacttaaattccccttggccttttccaggtcactaccctcttccgtcattactgccaggctctcgctatcttcctcctcaacgtcagggaatgagggctgggcattgccatccaggggttctgcgagagcattctgcgggtctttcctttctgtttcagaatcacacctgttctcacaagggataaatttgtcaccttcagtttttatttcaggaacttccaataggtcttttttatgatctgttaaaacatactttgggactctaggtggtttggtttcttctgagaagttggagccactgtcccagccattttctgcactttcagagttactttcattgtcatcagaggagcagaagggtggctgagaatcatcaatcttgtctcttccatcatcagaatgaatcagaaagcactcgtctgcttcatcgctctctgcttttaaagactggatgccactgtcatttaaattttcacttacagtctgaacagatacatttttttcaaatttccccaagtgcattaaagacttgaccatgagctcttgataacaagagtatctgtcttccttcctactggagttttcttgtgcagttgaaagaagactttcatccataggttttatcatgatttcctctgcggtagagtgaccatgtgtttccaaggggccatcgtcctctgtcctgtcactgcggtcttcttggcagtctgcttttgggctgtagtgtcggggcttcattagcagggatttccttttgttgactggaacccccaaagcctgatcttcagctgttctcttctttgccatggagcaatcataggcaacactgagctcctggattagtgaatccattggcacctcggttcctttagagcgagtacgcagcgttttatcttcagcctctgcatccataaacctataaacagatgtataaagtgatttcctagtacttgtacttgacgtcttttcttactggagcttacatcaggggcaataagcaggtctcttccacatcgccccagtgcacagatctggtaccttcttttaggctgaagaggaagtcctggaattgctctctttttctccaggtaacttgtatgtcaactcagtttgccctgctgtgtcagggggactaaataaatgactttgtcttatttagtgataaatcctgaaattcattctttcttgcagaaaatttctaccgtcctgccttctctaccctttgcagtatatcaaagtgctcagctttttaatcatagatttctgtgtttcttgtaggatttgaccagacattaaatagatgcttcttcaacttaagtcagcaactgtagttccttccctaaaagctactggatctgaactggagagtttccatcactcctttacctggcgaacgtctacaggtgtgtcgaaagttatcttttcctggatgtgttccaaaatgctcttatgctatttctcttaggatttctccacgctgccccattcagaaattttattattttcttccacaactctgccaggcactggtttttgcgtgggatgatgccagcttctctcttcatgtggccttattaaaagccatggtttccgagatgtaaaacacccacagttacctcaattatttttctctccttacctctagtattcccctgaggtcacattcagttaaaaacatcctgcccttctccctacaaaaaggt

SEQ ID NO: 18669 - RNA, 4926 nt, Homo sapiens
  source 1..4926: mol_type = other RNA
tgagtgtgtgtgtgtgagtgtgtgtgtatattttgtagcatttgaagttttgtggcaagatttctatcaaattgaatgttgtcttgtttcctatggtgggtgagacccaaggtgccagtgtttgaagtaatcattcagattggagtagcattttttcatgtgttactatattttccattcctttccagtcaacccagtaagataaatgctatttcaggggatatggtatctacaaaatttttcatttggatgtgtttgtatttgctaagtacaaatctacaccaatattgtcacttgtatattgtaccaacatatggcaggaaagcctggctggtcacaccaagtcttatttttcatcttgggatacgagttgccaacgatctgatatgacttgaaaaacaaacagacaaatctgcatcactaaaaaggcttatgtttctttaaaacatttcaaataaataattcatattaacgaaaaccgtccagccaagtcgaatactttgctgattgctatatttaattattgctaacaaattctgagcaggctgttttccagcatcctgtgcttttgtgagtgcggattccccactagtgggcgccatttgtcttcttattccttccgtgcagctcaccttaccgcaaattcatttataaatacaaaaatcagtgaaaggtgggggaagaagtgtgcaataaaaatcaaactcaactatagtgcagtccttagacaaggatttccttcaccctttcctgtttcctcattaaaacccagcaagaaagatgacttgagaatagcatttctatttaaatcctattggaaaataaattaataaacacacttgtaaaaatacggcagacttcaaaatgcagttaaaagataaaaaactctttgattagtaataaataaattataaaaatgtcacatttattttacatatactttacaaaaaaaaaaagagtacaatgaagaaataaaagaaaaacatatgaaaataaataagatctaataattgactgcattgcttttaatccaagaagtctatcatagtttttctttcctttttatatcagctggggaaaataaaattagtgcaatgttgcaaattgtaaatgcagtacggcaacctccacgccttagcagtacatgaacctctaacagatccatctggagtttactgctgttggtaacttctgttgcccggcagcgctgtgatcctacacatggatacccttcactgcctgtttgatactttccagtagagctttgcattccggggaatagtcccgttccagattgctgtacatatctgtgagtgtatttacatatgcttcaaaattctgctcactgataggtcccatctgtggaagctggatgtcagcaaggcttgaaatgagagcttggcttagacctgccagctctttcagcagactttcattgttctgttctatgagtttgttctcctcctctatcgtctttaagttgctctccatagatgtgatctgggtctgaagtttcatcatatctgcttcaattttaaggttggattcattcagttcctttatttcttcatccaaatgcctaatttcttcatcactctctattcccccagttgctttgagcttgatggtcatgagttcttcagaaaccttgccctttttgataacttgtgcattgagaggacatccagataagcttcggtgggtgacaaaaacattatttacatggcccagcccattgcagcctggcaagggacaatgtggtagctcttgtttgttcagtttccaggagagggaggctccattgagaggattctccttctgtctcttggcagccagaggacagccagaagctgtgcggtgtgatgtgtatttacctgatatgtgaccttggccatcacaccctatcacaggacatttcagttcagggtcttctttttcttccttggtaggggtcattttgacaccacctttccttgcacgagggcatccggacaagcttctgtgggaagcatagtttccagtcacgtgccccgagccatcgcagcctggggttggacacttaagctcctgagagttggcagccatgagggattttagagtcttatctgctaaaggacatccagaaacactgcgatgagatgcatagtttcctgtcacgtggccacttccatcacatcctggtgttggacaggtgattagttcctttttgagatctcttgcatgaagcttgggtttagggcttggtatagaggcctctccaggaaactttttttcctctaaattttctagagagctcactgggtctttctctttctcctcctctgtcttcccgtgagttttgctatagttgataggagtgtcccagccctcttggtcacaaagagcctgatagaatgctgcattgaccagaatgctgcttgttttgaatggggaagaggaaggagttggaatagaagtgttagaggaagttaggggtgcagacttgtccaggattcgattttttttcatgcttaagtccaatgtgccattttcatccacttctatttcggctcccttggcatgcagactctgtggcttgttggagaggatgtctgtggcttccctgcagcgggtggaaaggttcaggatggcagcagctgctgctatgtgggtgtcttcactacattgaccgtagctataagagctggcacggccagggctctgggtgtgggcgcctgcactaggcagtcgattaggaaatttcactggatttggaaaatgctttgattcaggaaatggtggtgtttttcgtccttgcactgtttgtatgagagggcgtttaccgaaaacttgggcatcaaaactggcataatcaaatggtacttttccaaacttctcttgttcttttgacactgtggctctgggagaggtgatggcttgtgacgggaaattgaattcaatttgcttcaccaaacttgtcctgtgggcctggtcaggacactgcccagtttggggagaatcaagctgatttttatcctgggacattgccaatttttcagctgcagcaattggacaaccagaaagactcctgtgggtgttgcggttgctgttcacatgaccccttcctgtgcatcccggcgtgggacacttgagcacattttcatgcatggcaagaatttccaggggaacccgcactttgtgggggcaccccgaaaggctgcggtggtgcgggtagagccctgtcacgtgtcccgtgccatcacatccagggatcgggcacttggtctccctcttttcaggccttggtgaatgtttattgttaaagatttgtcttccacccatgtcgataactttggtttgcctcctttcccctgctaggtgctccagcaggaacctatccagctctttgtaggtgttatggaaaacacaacctcgctcagcctgcagagcaattgcctgctccagcaaacttaaattccccttggccttttccaggtcactaccctcttccgtcattactgccaggctctcgctatcttcctcctcaacgtcagggaatgagggctgggcattgccatccaggggttctgcgagagcattctgcgggtctttcctttctgtttcagaatcacacctgttctcacaagggataaatttgtcaccttcagtttttatttcaggaacttccaataggtcttttttatgatctgttaaaacatactttgggactctaggtggtttggtttcttctgagaagttggagccactgtcccagccattttctgcactttcagagttactttcattgtcatcagaggagcagaagggtggctgagaatcatcaatcttgtctcttccatcatcagaatgaatcagaaagcactcgtctgcttcatcgctctctgcttttaaagactggatgccactgtcatttaaattttcacttacagtctgaacagatacatttttttcaaatttccccaagtgcattaaagacttgaccatgagctcttgataacaagagtatctgtcttccttcctactggagttttcttgtgcagttgaaagaagactttcatccataggttttatcatgatttcctctgcggtagagtgaccatgtgtttccaaggggccatcgtcctctgtcctgtcactgcggtcttcttggcagtctgcttttgggctgtagtgtcggggcttcattagcagggatttccttttgttgactggaacccccaaagcctgatcttcagctgttctcttctttgccatggagcaatcataggcaacactgagctcctggattagtgaatccattggcacctcggttcctttagagcgagtacgcagcgttttatcttcagcctctgcatccataaacctataaacagatgtataaagtgatttcctagtacttgtacttgacgtcttttcttactggagcttacatcaggggcaataagcaggtctcttccacatcgccccagtgcacagatctggtaccttcttttaggctgaagaggaagtcctggaattgctctctttttctccaggtaacttgtatgtcaactcagtttgccctgctgtgtcagggggactaaataaatgactttgtcttatttagtgataaatcctgaaattcattctttcttgcagaaaatttctaccgtcctgccttctctaccctttgcagtatatcaaagtgctcagctttttaatcatagatttctgtgtttcttgtaggatttgaccagacattaaatagatgcttcttcaacttaagtcagcaactgtagttccttccctaaaagctactggatctgaactggagagtttccatcactcttttttgtttgtttccaaaacttatatttctctcctccctggtgggctgaacggaaacactaaagctgtttctttgaaaggtagttcccatgatatgac

SEQ ID NO: 18670 - RNA, 4934 nt, Homo sapiens
  source 1..4934: mol_type = other RNA
tgagtgtgtgtgtgtgagtgtgtgtgtatattttgtagcatttgaagttttgtggcaagatttctatcaaattgaatgttgtcttgtttcctatggtgggtgagacccaaggtgccagtgtttgaagtaatcattcagattggagtagcattttttcatgtgttactatattttccattcctttccagtcaacccagtaagataaatgctatttcaggggatatggtatctacaaaatttttcatttggatgtgtttgtatttgctaagtacaaatctacaccaatattgtcacttgtatattgtaccaacatatggcaggaaagcctggctggtcacaccaagtcttatttttcatcttgggatacgagttgccaacgatctgatatgacttgaaaaacaaacagacaaatctgcatcactaaaaaggcttatgtttctttaaaacatttcaaataaataattcatattaacgaaaaccgtccagccaagtcgaatactttgctgattgctatatttaattattgctaacaaattctgagcaggctgttttccagcatcctgtgcttttgtgagtgcggattccccactagtgggcgccatttgtcttcttattccttccgtgcagctcaccttaccgcaaattcatttataaatacaaaaatcagtgaaaggtgggggaagaagtgtgcaataaaaatcaaactcaactatagtgcagtccttagacaaggatttccttcaccctttcctgtttcctcattaaaacccagcaagaaagatgacttgagaatagcatttctatttaaatcctattggaaaataaattaataaacacacttgtaaaaatacggcagacttcaaaatgcagttaaaagataaaaaactctttgattagtaataaataaattataaaaatgtcacatttattttacatatactttacaaaaaaaaaaagagtacaatgaagaaataaaagaaaaacatatgaaaataaataagatctaataattgactgcattgcttttaatccaagaagtctatcatagtttttctttcctttttatatcagctggggaaaataaaattagtgcaatgttgcaaattgtaaatgcagtacggcaacctccacgccttagcagtacatgaacctctaacagatccatctggagtttactgctgttggtaacttctgttgcccggcagcgctgtgatcctacacatggatacccttcactgcctgtttgatactttccagtagagctttgcattccggggaatagtcccgttccagattgctgtacatatctgtgagtgtatttacatatgcttcaaaattctgctcactgataggtcccatctgtggaagctggatgtcagcaaggcttgaaatgagagcttggcttagacctgccagctctttcagcagactttcattgttctgttctatgagtttgttctcctcctctatcgtctttaagttgctctccatagatgtgatctgggtctgaagtttcatcatatctgcttcaattttaaggttggattcattcagttcctttatttcttcatccaaatgcctaatttcttcatcactctctattcccccagttgctttgagcttgatggtcatgagttcttcagaaaccttgccctttttgataacttgtgcattgagaggacatccagataagcttcggtgggtgacaaaaacattatttacatggcccagcccattgcagcctggcaagggacaatgtggtagctcttgtttgttcagtttccaggagagggaggctccattgagaggattctccttctgtctcttggcagccagaggacagccagaagctgtgcggtgtgatgtgtatttacctgatatgtgaccttggccatcacaccctatcacaggacatttcagttcagggtcttctttttcttccttggtaggggtcattttgacaccacctttccttgcacgagggcatccggacaagcttctgtgggaagcatagtttccagtcacgtgccccgagccatcgcagcctggggttggacacttaagctcctgagagttggcagccatgagggattttagagtcttatctgctaaaggacatccagaaacactgcgatgagatgcatagtttcctgtcacgtggccacttccatcacatcctggtgttggacaggtgattagttcctttttgagatctcttgcatgaagcttgggtttagggcttggtatagaggcctctccaggaaactttttttcctctaaattttctagagagctcactgggtctttctctttctcctcctctgtcttcccgtgagttttgctatagttgataggagtgtcccagccctcttggtcacaaagagcctgatagaatgctgcattgaccagaatgctgcttgttttgaatggggaagaggaaggagttggaatagaagtgttagaggaagttaggggtgcagacttgtccaggattcgattttttttcatgcttaagtccaatgtgccattttcatccacttctatttcggctcccttggcatgcagactctgtggcttgttggagaggatgtctgtggcttccctgcagcgggtggaaaggttcaggatggcagcagctgctgctatgtgggtgtcttcactacattgaccgtagctataagagctggcacggccagggctctgggtgtgggcgcctgcactaggcagtcgattaggaaatttcactggatttggaaaatgctttgattcaggaaatggtggtgtttttcgtccttgcactgtttgtatgagagggcgtttaccgaaaacttgggcatcaaaactggcataatcaaatggtacttttccaaacttctcttgttcttttgacactgtggctctgggagaggtgatggcttgtgacgggaaattgaattcaatttgcttcaccaaacttgtcctgtgggcctggtcaggacactgcccagtttggggagaatcaagctgatttttatcctgggacattgccaatttttcagctgcagcaattggacaaccagaaagactcctgtgggtgttgcggttgctgttcacatgaccccttcctgtgcatcccggcgtgggacacttgagcacattttcatgcatggcaagaatttccaggggaacccgcactttgtgggggcaccccgaaaggctgcggtggtgcgggtagagccctgtcacgtgtcccgtgccatcacatccagggatcgggcacttggtctccctcttttcaggccttggtgaatgtttattgttaaagatttgtcttccacccatgtcgataactttggtttgcctcctttcccctgctaggtgctccagcaggaacctatccagctctttgtaggtgttatggaaaacacaacctcgctcagcctgcagagcaattgcctgctccagcaaacttaaattccccttggccttttccaggtcactaccctcttccgtcattactgccaggctctcgctatcttcctcctcaacgtcagggaatgagggctgggcattgccatccaggggttctgcgagagcattctgcgggtctttcctttctgtttcagaatcacacctgttctcacaagggataaatttgtcaccttcagtttttatttcaggaacttccaataggtcttttttatgatctgttaaaacatactttgggactctaggtggtttggtttcttctgagaagttggagccactgtcccagccattttctgcactttcagagttactttcattgtcatcagaggagcagaagggtggctgagaatcatcaatcttgtctcttccatcatcagaatgaatcagaaagcactcgtctgcttcatcgctctctgcttttaaagactggatgccactgtcatttaaattttcacttacagtctgaacagatacatttttttcaaatttccccaagtgcattaaagacttgaccatgagctcttgataacaagagtatctgtcttccttcctactggagttttcttgtgcagttgaaagaagactttcatccataggttttatcatgatttcctctgcggtagagtgaccatgtgtttccaaggggccatcgtcctctgtcctgtcactgcggtcttcttggcagtctgcttttgggctgtagtgtcggggcttcattagcagggatttccttttgttgactggaacccccaaagcctgatcttcagctgttctcttctttgccatggagcaatcataggcaacactgagctcctggattagtgaatccattggcacctcggttcctttagagcgagtacgcagcgttttatcttcagcctctgcatccatatcaggggcaataagcaggtctcttccacatcgccccagtgcacagatctggtaccttcttttaggctgaagaggaagtcctggaattgctctctttttctccaggtaacttgtatgtcaactcagtttgccctgctgtgtcagggggactaaataaatgactttgtcttatttagtgataaatcctgaaattcattctttcttgcagaaaatttctaccgtcctgccttctctaccctttgcagtatatcaaagtgctcagctttttaatcatagatttctgtgtttcttgtaggatttgaccagacattaaatagatgcttcttcaacttaagtcagcaactgtagttccttccctaaaagctactggatctgaactggagagtttccatcactccttagtcttgatatgagcacgcagacacataaaatggaattgtcacaatgcttcagggacactcacaaaattgggggctttttttgtttgtttccaaaacttatatttctctcctccctggtgggctgaacggaaacactaaagctgtttctttgaaaggtagttcccatgatatgac

SEQ ID NO: 18671 - RNA, 4956 nt, Homo sapiens
  source 1..4956: mol_type = other RNA
tgagtgtgtgtgtgtgagtgtgtgtgtatattttgtagcatttgaagttttgtggcaagatttctatcaaattgaatgttgtcttgtttcctatggtgggtgagacccaaggtgccagtgtttgaagtaatcattcagattggagtagcattttttcatgtgttactatattttccattcctttccagtcaacccagtaagataaatgctatttcaggggatatggtatctacaaaatttttcatttggatgtgtttgtatttgctaagtacaaatctacaccaatattgtcacttgtatattgtaccaacatatggcaggaaagcctggctggtcacaccaagtcttatttttcatcttgggatacgagttgccaacgatctgatatgacttgaaaaacaaacagacaaatctgcatcactaaaaaggcttatgtttctttaaaacatttcaaataaataattcatattaacgaaaaccgtccagccaagtcgaatactttgctgattgctatatttaattattgctaacaaattctgagcaggctgttttccagcatcctgtgcttttgtgagtgcggattccccactagtgggcgccatttgtcttcttattccttccgtgcagctcaccttaccgcaaattcatttataaatacaaaaatcagtgaaaggtgggggaagaagtgtgcaataaaaatcaaactcaactatagtgcagtccttagacaaggatttccttcaccctttcctgtttcctcattaaaacccagcaagaaagatgacttgagaatagcatttctatttaaatcctattggaaaataaattaataaacacacttgtaaaaatacggcagacttcaaaatgcagttaaaagataaaaaactctttgattagtaataaataaattataaaaatgtcacatttattttacatatactttacaaaaaaaaaaagagtacaatgaagaaataaaagaaaaacatatgaaaataaataagatctaataattgactgcattgcttttaatccaagaagtctatcatagtttttctttcctttttatatcagctggggaaaataaaattagtgcaatgttgcaaattgtaaatgcagtacggcaacctccacgccttagcagtacatgaacctctaacagatccatctggagtttactgctgttggtaacttctgttgcccggcagcgctgtgatcctacacatggatacccttcactgcctgtttgatactttccagtagagctttgcattccggggaatagtcccgttccagattgctgtacatatctgtgagtgtatttacatatgcttcaaaattctgctcactgataggtcccatctgtggaagctggatgtcagcaaggcttgaaatgagagcttggcttagacctgccagctctttcagcagactttcattgttctgttctatgagtttgttctcctcctctatcgtctttaagttgctctccatagatgtgatctgggtctgaagtttcatcatatctgcttcaattttaaggttggattcattcagttcctttatttcttcatccaaatgcctaatttcttcatcactctctattcccccagttgctttgagcttgatggtcatgagttcttcagaaaccttgccctttttgataacttgtgcattgagaggacatccagataagcttcggtgggtgacaaaaacattatttacatggcccagcccattgcagcctggcaagggacaatgtggtagctcttgtttgttcagtttccaggagagggaggctccattgagaggattctccttctgtctcttggcagccagaggacagccagaagctgtgcggtgtgatgtgtatttacctgatatgtgaccttggccatcacaccctatcacaggacatttcagttcagggtcttctttttcttccttggtaggggtcattttgacaccacctttccttgcacgagggcatccggacaagcttctgtgggaagcatagtttccagtcacgtgccccgagccatcgcagcctggggttggacacttaagctcctgagagttggcagccatgagggattttagagtcttatctgctaaaggacatccagaaacactgcgatgagatgcatagtttcctgtcacgtggccacttccatcacatcctggtgttggacaggtgattagttcctttttgagatctcttgcatgaagcttgggtttagggcttggtatagaggcctctccaggaaactttttttcctctaaattttctagagagctcactgggtctttctctttctcctcctctgtcttcccgtgagttttgctatagttgataggagtgtcccagccctcttggtcacaaagagcctgatagaatgctgcattgaccagaatgctgcttgttttgaatggggaagaggaaggagttggaatagaagtgttagaggaagttaggggtgcagacttgtccaggattcgattttttttcatgcttaagtccaatgtgccattttcatccacttctatttcggctcccttggcatgcagactctgtggcttgttggagaggatgtctgtggcttccctgcagcgggtggaaaggttcaggatggcagcagctgctgctatgtgggtgtcttcactacattgaccgtagctataagagctggcacggccagggctctgggtgtgggcgcctgcactaggcagtcgattaggaaatttcactggatttggaaaatgctttgattcaggaaatggtggtgtttttcgtccttgcactgtttgtatgagagggcgtttaccgaaaacttgggcatcaaaactggcataatcaaatggtacttttccaaacttctcttgttcttttgacactgtggctctgggagaggtgatggcttgtgacgggaaattgaattcaatttgcttcaccaaacttgtcctgtgggcctggtcaggacactgcccagtttggggagaatcaagctgatttttatcctgggacattgccaatttttcagctgcagcaattggacaaccagaaagactcctgtgggtgttgcggttgctgttcacatgaccccttcctgtgcatcccggcgtgggacacttgagcacattttcatgcatggcaagaatttccaggggaacccgcactttgtgggggcaccccgaaaggctgcggtggtgcgggtagagccctgtcacgtgtcccgtgccatcacatccagggatcgggcacttggtctccctcttttcaggccttggtgaatgtttattgttaaagatttgtcttccacccatgtcgataactttggtttgcctcctttcccctgctaggtgctccagcaggaacctatccagctctttgtaggtgttatggaaaacacaacctcgctcagcctgcagagcaattgcctgctccagcaaacttaaattccccttggccttttccaggtcactaccctcttccgtcattactgccaggctctcgctatcttcctcctcaacgtcagggaatgagggctgggcattgccatccaggggttctgcgagagcattctgcgggtctttcctttctgtttcagaatcacacctgttctcacaagggataaatttgtcaccttcagtttttatttcaggaacttccaataggtcttttttatgatctgttaaaacatactttgggactctaggtggtttggtttcttctgagaagttggagccactgtcccagccattttctgcactttcagagttactttcattgtcatcagaggagcagaagggtggctgagaatcatcaatcttgtctcttccatcatcagaatgaatcagaaagcactcgtctgcttcatcgctctctgcttttaaagactggatgccactgtcatttaaattttcacttacagtctgaacagatacatttttttcaaatttccccaagtgcattaaagacttgaccatgagctcttgataacaagagtatctgtcttccttcctactggagttttcttgtgcagttgaaagaagactttcatccataggttttatcatgatttcctctgcggtagagtgaccatgtgtttccaaggggccatcgtcctctgtcctgtcactgcggtcttcttggcagtctgcttttgggctgtagtgtcggggcttcattagcagggatttccttttgttgactggaacccccaaagcctgatcttcagctgttctcttctttgccatggagcaatcataggcaacactgagctcctggattagtgaatccattggcacctcggttcctttagagcgagtacgcagcgttttatcttcagcctctgcatccatatcaggggcaataagcaggtctcttccacatcgccccagtgcacagatctggtaccttcttttaggctgaagaggaagtcctggaattgctctctttttctccaggtaacttgtatgtcaactcagtttgccctgctgtgtcagggggactaaataaatgactttgtcttatttagtgataaatcctgaaattcattctttcttgcagaaaatttctaccgtcctgccttctctaccctttgcagtatatcaaagtgctcagctttttaatcatagatttctgtgtttcttgtaggatttgaccagacattaaatagatgcttcttcaacttaagtcagcaactgtagttccttccctaaaagctactggatctgaactggagagtttccatcactcctttacctggcgaacgtctacaggtgtgtcgaaagttatcttttcctggatgtgttccaaaatgctcttatgctatttctcttaggatttctccacgctgccccattcagaaattttattattttctctagtattcccctgaggtcacattcagttaaaaacatcctgcccttctccctacaaaaaggttccatagaatc

SEQ ID NO: 18672 - RNA, 4948 nt, Homo sapiens
  source 1..4948: mol_type = other RNA
tgagtgtgtgtgtgtgagtgtgtgtgtatattttgtagcatttgaagttttgtggcaagatttctatcaaattgaatgttgtcttgtttcctatggtgggtgagacccaaggtgccagtgtttgaagtaatcattcagattggagtagcattttttcatgtgttactatattttccattcctttccagtcaacccagtaagataaatgctatttcaggggatatggtatctacaaaatttttcatttggatgtgtttgtatttgctaagtacaaatctacaccaatattgtcacttgtatattgtaccaacatatggcaggaaagcctggctggtcacaccaagtcttatttttcatcttgggatacgagttgccaacgatctgatatgacttgaaaaacaaacagacaaatctgcatcactaaaaaggcttatgtttctttaaaacatttcaaataaataattcatattaacgaaaaccgtccagccaagtcgaatactttgctgattgctatatttaattattgctaacaaattctgagcaggctgttttccagcatcctgtgcttttgtgagtgcggattccccactagtgggcgccatttgtcttcttattccttccgtgcagctcaccttaccgcaaattcatttataaatacaaaaatcagtgaaaggtgggggaagaagtgtgcaataaaaatcaaactcaactatagtgcagtccttagacaaggatttccttcaccctttcctgtttcctcattaaaacccagcaagaaagatgacttgagaatagcatttctatttaaatcctattggaaaataaattaataaacacacttgtaaaaatacggcagacttcaaaatgcagttaaaagataaaaaactctttgattagtaataaataaattataaaaatgtcacatttattttacatatactttacaaaaaaaaaaagagtacaatgaagaaataaaagaaaaacatatgaaaataaataagatctaataattgactgcattgcttttaatccaagaagtctatcatagtttttctttcctttttatatcagctggggaaaataaaattagtgcaatgttgcaaattgtaaatgcagtacggcaacctccacgccttagcagtacatgaacctctaacagatccatctggagtttactgctgttggtaacttctgttgcccggcagcgctgtgatcctacacatggatacccttcactgcctgtttgatactttccagtagagctttgcattccggggaatagtcccgttccagattgctgtacatatctgtgagtgtatttacatatgcttcaaaattctgctcactgataggtcccatctgtggaagctggatgtcagcaaggcttgaaatgagagcttggcttagacctgccagctctttcagcagactttcattgttctgttctatgagtttgttctcctcctctatcgtctttaagttgctctccatagatgtgatctgggtctgaagtttcatcatatctgcttcaattttaaggttggattcattcagttcctttatttcttcatccaaatgcctaatttcttcatcactctctattcccccagttgctttgagcttgatggtcatgagttcttcagaaaccttgccctttttgataacttgtgcattgagaggacatccagataagcttcggtgggtgacaaaaacattatttacatggcccagcccattgcagcctggcaagggacaatgtggtagctcttgtttgttcagtttccaggagagggaggctccattgagaggattctccttctgtctcttggcagccagaggacagccagaagctgtgcggtgtgatgtgtatttacctgatatgtgaccttggccatcacaccctatcacaggacatttcagttcagggtcttctttttcttccttggtaggggtcattttgacaccacctttccttgcacgagggcatccggacaagcttctgtgggaagcatagtttccagtcacgtgccccgagccatcgcagcctggggttggacacttaagctcctgagagttggcagccatgagggattttagagtcttatctgctaaaggacatccagaaacactgcgatgagatgcatagtttcctgtcacgtggccacttccatcacatcctggtgttggacaggtgattagttcctttttgagatctcttgcatgaagcttgggtttagggcttggtatagaggcctctccaggaaactttttttcctctaaattttctagagagctcactgggtctttctctttctcctcctctgtcttcccgtgagttttgctatagttgataggagtgtcccagccctcttggtcacaaagagcctgatagaatgctgcattgaccagaatgctgcttgttttgaatggggaagaggaaggagttggaatagaagtgttagaggaagttaggggtgcagacttgtccaggattcgattttttttcatgcttaagtccaatgtgccattttcatccacttctatttcggctcccttggcatgcagactctgtggcttgttggagaggatgtctgtggcttccctgcagcgggtggaaaggttcaggatggcagcagctgctgctatgtgggtgtcttcactacattgaccgtagctataagagctggcacggccagggctctgggtgtgggcgcctgcactaggcagtcgattaggaaatttcactggatttggaaaatgctttgattcaggaaatggtggtgtttttcgtccttgcactgtttgtatgagagggcgtttaccgaaaacttgggcatcaaaactggcataatcaaatggtacttttccaaacttctcttgttcttttgacactgtggctctgggagaggtgatggcttgtgacgggaaattgaattcaatttgcttcaccaaacttgtcctgtgggcctggtcaggacactgcccagtttggggagaatcaagctgatttttatcctgggacattgccaatttttcagctgcagcaattggacaaccagaaagactcctgtgggtgttgcggttgctgttcacatgaccccttcctgtgcatcccggcgtgggacacttgagcacattttcatgcatggcaagaatttccaggggaacccgcactttgtgggggcaccccgaaaggctgcggtggtgcgggtagagccctgtcacgtgtcccgtgccatcacatccagggatcgggcacttggtctccctcttttcaggccttggtgaatgtttattgttaaagatttgtcttccacccatgtcgataactttggtttgcctcctttcccctgctaggtgctccagcaggaacctatccagctctttgtaggtgttatggaaaacacaacctcgctcagcctgcagagcaattgcctgctccagcaaacttaaattccccttggccttttccaggtcactaccctcttccgtcattactgccaggctctcgctatcttcctcctcaacgtcagggaatgagggctgggcattgccatccaggggttctgcgagagcattctgcgggtctttcctttctgtttcagaatcacacctgttctcacaagggataaatttgtcaccttcagtttttatttcaggaacttccaataggtcttttttatgatctgttaaaacatactttgggactctaggtggtttggtttcttctgagaagttggagccactgtcccagccattttctgcactttcagagttactttcattgtcatcagaggagcagaagggtggctgagaatcatcaatcttgtctcttccatcatcagaatgaatcagaaagcactcgtctgcttcatcgctctctgcttttaaagactggatgccactgtcatttaaattttcacttacagtctgaacagatacatttttttcaaatttccccaagtgcattaaagacttgaccatgagctcttgataacaagagtatctgtcttccttcctactggagttttcttgtgcagttgaaagaagactttcatccataggttttatcatgatttcctctgcggtagagtgaccatgtgtttccaaggggccatcgtcctctgtcctgtcactgcggtcttcttggcagtctgcttttgggctgtagtgtcggggcttcattagcagggatttccttttgttgactggaacccccaaagcctgatcttcagctgttctcttctttgccatggagcaatcataggcaacactgagctcctggattagtgaatccattggcacctcggttcctttagagcgagtacgcagcgttttatcttcagcctctgcatccatctataaacagatgtataaagtgatttcctagtacttgtacttgacgtcttttcttactggagcttacatcaggggcaataagcaggtctcttccacatcgccccagtgcacagatctggtaccttcttttaggctgaagaggaagtcctggaattgctctctttttctccaggtaacttgtatgtcaactcagtttgccctgctgtgtcagggggactaaataaatgactttgtcttatttagtgataaatcctgaaattcattcttccctaaaagctactggatctgaactggagagtttccatcactccttagtcttgatatgagcacgcagacacataaaatggaattgtcacaatgcttcagggacactcacaaaattgggggctctttacctggcgaacgtctacaggtgtgtcgaaagttatcttttcctggatgtgttccaaaatgctcttatgctatttctcttaggatttctccacgctgccccattcagaaattttattattttctctagtattcccctgaggtcacattcagttaaaaacatcctgcccttctccctacaaaaaggttccatagaatc

SEQ ID NO: 18673 - RNA, 5277 nt, Homo sapiens
  source 1..5277: mol_type = other RNA
tgagtgtgtgtgtgtgagtgtgtgtgtatattttgtagcatttgaagttttgtggcaagatttctatcaaattgaatgttgtcttgtttcctatggtgggtgagacccaaggtgccagtgtttgaagtaatcattcagattggagtagcattttttcatgtgttactatattttccattcctttccagtcaacccagtaagataaatgctatttcaggggatatggtatctacaaaatttttcatttggatgtgtttgtatttgctaagtacaaatctacaccaatattgtcacttgtatattgtaccaacatatggcaggaaagcctggctggtcacaccaagtcttatttttcatcttgggatacgagttgccaacgatctgatatgacttgaaaaacaaacagacaaatctgcatcactaaaaaggcttatgtttctttaaaacatttcaaataaataattcatattaacgaaaaccgtccagccaagtcgaatactttgctgattgctatatttaattattgctaacaaattctgagcaggctgttttccagcatcctgtgcttttgtgagtgcggattccccactagtgggcgccatttgtcttcttattccttccgtgcagctcaccttaccgcaaattcatttataaatacaaaaatcagtgaaaggtgggggaagaagtgtgcaataaaaatcaaactcaactatagtgcagtccttagacaaggatttccttcaccctttcctgtttcctcattaaaacccagcaagaaagatgacttgagaatagcatttctatttaaatcctattggaaaataaattaataaacacacttgtaaaaatacggcagacttcaaaatgcagttaaaagataaaaaactctttgattagtaataaataaattataaaaatgtcacatttattttacatatactttacaaaaaaaaaaagagtacaatgaagaaataaaagaaaaacatatgaaaataaataagatctaataattgactgcattgcttttaatccaagaagtctatcatagtttttctttcctttttatatcagctggggaaaataaaattagtgcaatgttgcaaattgtaaatgcagtacggcaacctccacgccttagcagtacatgaacctctaacagatccatctggagtttactgctgttggtaacttctgttgcccggcagcgctgtgatcctacacatggatacccttcactgcctgtttgatactttccagtagagctttgcattccggggaatagtcccgttccagattgctgtacatatctgtgagtgtatttacatatgcttcaaaattctgctcactgataggtcccatctgtggaagctggatgtcagcaaggcttgaaatgagagcttggcttagacctgccagctctttcagcagactttcattgttctgttctatgagtttgttctcctcctctatcgtctttaagttgctctccatagatgtgatctgggtctgaagtttcatcatatctgcttcaattttaaggttggattcattcagttcctttatttcttcatccaaatgcctaatttcttcatcactctctattcccccagttgctttgagcttgatggtcatgagttcttcagaaaccttgccctttttgataacttgtgcattgagaggacatccagataagcttcggtgggtgacaaaaacattatttacatggcccagcccattgcagcctggcaagggacaatgtggtagctcttgtttgttcagtttccaggagagggaggctccattgagaggattctccttctgtctcttggcagccagaggacagccagaagctgtgcggtgtgatgtgtatttacctgatatgtgaccttggccatcacaccctatcacaggacatttcagttcagggtcttctttttcttccttggtaggggtcattttgacaccacctttccttgcacgagggcatccggacaagcttctgtgggaagcatagtttccagtcacgtgccccgagccatcgcagcctggggttggacacttaagctcctgagagttggcagccatgagggattttagagtcttatctgctaaaggacatccagaaacactgcgatgagatgcatagtttcctgtcacgtggccacttccatcacatcctggtgttggacaggtgattagttcctttttgagatctcttgcatgaagcttgggtttagggcttggtatagaggcctctccaggaaactttttttcctctaaattttctagagagctcactgggtctttctctttctcctcctctgtcttcccgtgagttttgctatagttgataggagtgtcccagccctcttggtcacaaagagcctgatagaatgctgcattgaccagaatgctgcttgttttgaatggggaagaggaaggagttggaatagaagtgttagaggaagttaggggtgcagacttgtccaggattcgattttttttcatgcttaagtccaatgtgccattttcatccacttctatttcggctcccttggcatgcagactctgtggcttgttggagaggatgtctgtggcttccctgcagcgggtggaaaggttcaggatggcagcagctgctgctatgtgggtgtcttcactacattgaccgtagctataagagctggcacggccagggctctgggtgtgggcgcctgcactaggcagtcgattaggaaatttcactggatttggaaaatgctttgattcaggaaatggtggtgtttttcgtccttgcactgtttgtatgagagggcgtttaccgaaaacttgggcatcaaaactggcataatcaaatggtacttttccaaacttctcttgttcttttgacactgtggctctgggagaggtgatggcttgtgacgggaaattgaattcaatttgcttcaccaaacttgtcctgtgggcctggtcaggacactgcccagtttggggagaatcaagctgatttttatcctgggacattgccaatttttcagctgcagcaattggacaaccagaaagactcctgtgggtgttgcggttgctgttcacatgaccccttcctgtgcatcccggcgtgggacacttgagcacattttcatgcatggcaagaatttccaggggaacccgcactttgtgggggcaccccgaaaggctgcggtggtgcgggtagagccctgtcacgtgtcccgtgccatcacatccagggatcgggcacttggtctccctcttttcaggccttggtgaatgtttattgttaaagatttgtcttccacccatgtcgataactttggtttgcctcctttcccctgctaggtgctccagcaggaacctatccagctctttgtaggtgttatggaaaacacaacctcgctcagcctgcagagcaattgcctgctccagcaaacttaaattccccttggccttttccaggtcactaccctcttccgtcattactgccaggctctcgctatcttcctcctcaacgtcagggaatgagggctgggcattgccatccaggggttctgcgagagcattctgcgggtctttcctttctgtttcagaatcacacctgttctcacaagggataaatttgtcaccttcagtttttatttcaggaacttccaataggtcttttttatgatctgttaaaacatactttgggactctaggtggtttggtttcttctgagaagttggagccactgtcccagccattttctgcactttcagagttactttcattgtcatcagaggagcagaagggtggctgagaatcatcaatcttgtctcttccatcatcagaatgaatcagaaagcactcgtctgcttcatcgctctctgcttttaaagactggatgccactgtcatttaaattttcacttacagtctgaacagatacatttttttcaaatttccccaagtgcattaaagacttgaccatgagctcttgataacaagagtatctgtcttccttcctactggagttttcttgtgcagttgaaagaagactttcatccataggttttatcatgatttcctctgcggtagagtgaccatgtgtttccaaggggccatcgtcctctgtcctgtcactgcggtcttcttggcagtctgcttttgggctgtagtgtcggggcttcattagcagggatttccttttgttgactggaacccccaaagcctgatcttcagctgttctcttctttgccatggagcaatcataggcaacactgagctcctggattagtgaatccattggcacctcggttcctttagagcgagtacgcagcgttttatcttcagcctctgcatccatctataaacagatgtataaagtgatttcctagtacttgtacttgacgtcttttcttactggagcttacatcaggggcaataagcaggtctcttccacatcgccccagtgcacagatctggtaccttcttttaggctgaagaggaagtcctggaattgctctctttttctccaggtaacttgtatgtcaactcagtttgccctgctgtgtcagggggactaaataaatgactttgtcttatttagtgataaatcctgaaattcattctttcttgcagaaaatttctaccgtcctgccttctctaccctttgcagtatatcaaagtgctcagctttttaatcatagatttctgtgtttcttgtaggatttgaccagacattaaatagatgcttcttcaacttaagtcagcaactgtagttcactagtaggcataacagtatttgtatttgtccttccagtcccttccctaaaagctactggatctgaactggagagtttccatcactccttagtcttgatatgagcacgcagacacataaaatggaattgtcacaatgcttcagggacactcacaaaattgggggctctttacctggcgaacgtctacaggtgtgtcgaaagttatcttttcctggatgtgttccaaaatgctcttatgctatttctcttaggatttctccacgctgccccattcagaaattttattattttcttccacaactctgccaggcactggtttttgcgtgggatgatgccagcttctctcttcatgtggccttattaaaagccatggtttccgagatgtaaaacacccacagttacctcaattatttttctctccttacctctagtattcccctgaggtcacattcagttaaaaacatcctgcccttctccctacaaaaaggttccatagaatc

SEQ ID NO: 18674 - RNA, 5042 nt, Homo sapiens
  source 1..5042: mol_type = other RNA
tgagtgtgtgtgtgtgagtgtgtgtgtatattttgtagcatttgaagttttgtggcaagatttctatcaaattgaatgttgtcttgtttcctatggtgggtgagacccaaggtgccagtgtttgaagtaatcattcagattggagtagcattttttcatgtgttactatattttccattcctttccagtcaacccagtaagataaatgctatttcaggggatatggtatctacaaaatttttcatttggatgtgtttgtatttgctaagtacaaatctacaccaatattgtcacttgtatattgtaccaacatatggcaggaaagcctggctggtcacaccaagtcttatttttcatcttgggatacgagttgccaacgatctgatatgacttgaaaaacaaacagacaaatctgcatcactaaaaaggcttatgtttctttaaaacatttcaaataaataattcatattaacgaaaaccgtccagccaagtcgaatactttgctgattgctatatttaattattgctaacaaattctgagcaggctgttttccagcatcctgtgcttttgtgagtgcggattccccactagtgggcgccatttgtcttcttattccttccgtgcagctcaccttaccgcaaattcatttataaatacaaaaatcagtgaaaggtgggggaagaagtgtgcaataaaaatcaaactcaactatagtgcagtccttagacaaggatttccttcaccctttcctgtttcctcattaaaacccagcaagaaagatgacttgagaatagcatttctatttaaatcctattggaaaataaattaataaacacacttgtaaaaatacggcagacttcaaaatgcagttaaaagataaaaaactctttgattagtaataaataaattataaaaatgtcacatttattttacatatactttacaaaaaaaaaaagagtacaatgaagaaataaaagaaaaacatatgaaaataaataagatctaataattgactgcattgcttttaatccaagaagtctatcatagtttttctttcctttttatatcagctggggaaaataaaattagtgcaatgttgcaaattgtaaatgcagtacggcaacctccacgccttagcagtacatgaacctctaacagatccatctggagtttactgctgttggtaacttctgttgcccggcagcgctgtgatcctacacatggatacccttcactgcctgtttgatactttccagtagagctttgcattccggggaatagtcccgttccagattgctgtacatatctgtgagtgtatttacatatgcttcaaaattctgctcactgataggtcccatctgtggaagctggatgtcagcaaggcttgaaatgagagcttggcttagacctgccagctctttcagcagactttcattgttctgttctatgagtttgttctcctcctctatcgtctttaagttgctctccatagatgtgatctgggtctgaagtttcatcatatctgcttcaattttaaggttggattcattcagttcctttatttcttcatccaaatgcctaatttcttcatcactctctattcccccagttgctttgagcttgatggtcatgagttcttcagaaaccttgccctttttgataacttgtgcattgagaggacatccagataagcttcggtgggtgacaaaaacattatttacatggcccagcccattgcagcctggcaagggacaatgtggtagctcttgtttgttcagtttccaggagagggaggctccattgagaggattctccttctgtctcttggcagccagaggacagccagaagctgtgcggtgtgatgtgtatttacctgatatgtgaccttggccatcacaccctatcacaggacatttcagttcagggtcttctttttcttccttggtaggggtcattttgacaccacctttccttgcacgagggcatccggacaagcttctgtgggaagcatagtttccagtcacgtgccccgagccatcgcagcctggggttggacacttaagctcctgagagttggcagccatgagggattttagagtcttatctgctaaaggacatccagaaacactgcgatgagatgcatagtttcctgtcacgtggccacttccatcacatcctggtgttggacaggtgattagttcctttttgagatctcttgcatgaagcttgggtttagggcttggtatagaggcctctccaggaaactttttttcctctaaattttctagagagctcactgggtctttctctttctcctcctctgtcttcccgtgagttttgctatagttgataggagtgtcccagccctcttggtcacaaagagcctgatagaatgctgcattgaccagaatgctgcttgttttgaatggggaagaggaaggagttggaatagaagtgttagaggaagttaggggtgcagacttgtccaggattcgattttttttcatgcttaagtccaatgtgccattttcatccacttctatttcggctcccttggcatgcagactctgtggcttgttggagaggatgtctgtggcttccctgcagcgggtggaaaggttcaggatggcagcagctgctgctatgtgggtgtcttcactacattgaccgtagctataagagctggcacggccagggctctgggtgtgggcgcctgcactaggcagtcgattaggaaatttcactggatttggaaaatgctttgattcaggaaatggtggtgtttttcgtccttgcactgtttgtatgagagggcgtttaccgaaaacttgggcatcaaaactggcataatcaaatggtacttttccaaacttctcttgttcttttgacactgtggctctgggagaggtgatggcttgtgacgggaaattgaattcaatttgcttcaccaaacttgtcctgtgggcctggtcaggacactgcccagtttggggagaatcaagctgatttttatcctgggacattgccaatttttcagctgcagcaattggacaaccagaaagactcctgtgggtgttgcggttgctgttcacatgaccccttcctgtgcatcccggcgtgggacacttgagcacattttcatgcatggcaagaatttccaggggaacccgcactttgtgggggcaccccgaaaggctgcggtggtgcgggtagagccctgtcacgtgtcccgtgccatcacatccagggatcgggcacttggtctccctcttttcaggccttggtgaatgtttattgttaaagatttgtcttccacccatgtcgataactttggtttgcctcctttcccctgctaggtgctccagcaggaacctatccagctctttgtaggtgttatggaaaacacaacctcgctcagcctgcagagcaattgcctgctccagcaaacttaaattccccttggccttttccaggtcactaccctcttccgtcattactgccaggctctcgctatcttcctcctcaacgtcagggaatgagggctgggcattgccatccaggggttctgcgagagcattctgcgggtctttcctttctgtttcagaatcacacctgttctcacaagggataaatttgtcaccttcagtttttatttcaggaacttccaataggtcttttttatgatctgttaaaacatactttgggactctaggtggtttggtttcttctgagaagttggagccactgtcccagccattttctgcactttcagagttactttcattgtcatcagaggagcagaagggtggctgagaatcatcaatcttgtctcttccatcatcagaatgaatcagaaagcactcgtctgcttcatcgctctctgcttttaaagactggatgccactgtcatttaaattttcacttacagtctgaacagatacatttttttcaaatttccccaagtgcattaaagacttgaccatgagctcttgataacaagagtatctgtcttccttcctactggagttttcttgtgcagttgaaagaagactttcatccataggttttatcatgatttcctctgcggtagagtgaccatgtgtttccaaggggccatcgtcctctgtcctgtcactgcggtcttcttggcagtctgcttttgggctgtagtgtcggggcttcattagcagggatttccttttgttgactggaacccccaaagcctgatcttcagctgttctcttctttgccatggagcaatcataggcaacactgagctcctggattagtgaatccattggcacctcggttcctttagagcgagtacgcagcgttttatcttcagcctctgcatccatctataaacagatgtataaagtgatttcctagtacttgtacttgacgtcttttcttactggagcttacatcaggggcaataagcaggtctcttccacatcgccccagtgcacagatctggtaccttcttttaggctgaagaggaagtcctggaattgctctctttttctccaggtaacttgtatgtcaactcagtttgccctgctgtgtcagggggactaaataaatgactttgtcttatttagtgataaatcctgaaattcattctttcttgcagaaaatttctaccgtcctgccttctctaccctttgcagtatatcaaagtgctcagctttttaatcatagatttctgtgtttcttgtaggatttgaccagacattaaatagatgcttcttcaacttaagtcagcaactgtagttcactagtaggcataacagtatttgtatttgtccttccagtcccttccctaaaagctactggatctgaactggagagtttccatcactccttagtcttgatatgagcacgcagacacataaaatggaattgtcacaatgcttcagggacactcacaaaattgggggctttttttgtttgtttccaaaacttatatttctctcctccctggtgggctgaacggaaacactaaagctgtttctttgaaaggtagttcccatgatatgac

SEQ ID NO: 18675 - RNA, 5079 nt, Homo sapiens
  source 1..5079: mol_type = other RNA
tgagtgtgtgtgtgtgagtgtgtgtgtatattttgtagcatttgaagttttgtggcaagatttctatcaaattgaatgttgtcttgtttcctatggtgggtgagacccaaggtgccagtgtttgaagtaatcattcagattggagtagcattttttcatgtgttactatattttccattcctttccagtcaacccagtaagataaatgctatttcaggggatatggtatctacaaaatttttcatttggatgtgtttgtatttgctaagtacaaatctacaccaatattgtcacttgtatattgtaccaacatatggcaggaaagcctggctggtcacaccaagtcttatttttcatcttgggatacgagttgccaacgatctgatatgacttgaaaaacaaacagacaaatctgcatcactaaaaaggcttatgtttctttaaaacatttcaaataaataattcatattaacgaaaaccgtccagccaagtcgaatactttgctgattgctatatttaattattgctaacaaattctgagcaggctgttttccagcatcctgtgcttttgtgagtgcggattccccactagtgggcgccatttgtcttcttattccttccgtgcagctcaccttaccgcaaattcatttataaatacaaaaatcagtgaaaggtgggggaagaagtgtgcaataaaaatcaaactcaactatagtgcagtccttagacaaggatttccttcaccctttcctgtttcctcattaaaacccagcaagaaagatgacttgagaatagcatttctatttaaatcctattggaaaataaattaataaacacacttgtaaaaatacggcagacttcaaaatgcagttaaaagataaaaaactctttgattagtaataaataaattataaaaatgtcacatttattttacatatactttacaaaaaaaaaaagagtacaatgaagaaataaaagaaaaacatatgaaaataaataagatctaataattgactgcattgcttttaatccaagaagtctatcatagtttttctttcctttttatatcagctggggaaaataaaattagtgcaatgttgcaaattgtaaatgcagtacggcaacctccacgccttagcagtacatgaacctctaacagatccatctggagtttactgctgttggtaacttctgttgcccggcagcgctgtgatcctacacatggatacccttcactgcctgtttgatactttccagtagagctttgcattccggggaatagtcccgttccagattgctgtacatatctgtgagtgtatttacatatgcttcaaaattctgctcactgataggtcccatctgtggaagctggatgtcagcaaggcttgaaatgagagcttggcttagacctgccagctctttcagcagactttcattgttctgttctatgagtttgttctcctcctctatcgtctttaagttgctctccatagatgtgatctgggtctgaagtttcatcatatctgcttcaattttaaggttggattcattcagttcctttatttcttcatccaaatgcctaatttcttcatcactctctattcccccagttgctttgagcttgatggtcatgagttcttcagaaaccttgccctttttgataacttgtgcattgagaggacatccagataagcttcggtgggtgacaaaaacattatttacatggcccagcccattgcagcctggcaagggacaatgtggtagctcttgtttgttcagtttccaggagagggaggctccattgagaggattctccttctgtctcttggcagccagaggacagccagaagctgtgcggtgtgatgtgtatttacctgatatgtgaccttggccatcacaccctatcacaggacatttcagttcagggtcttctttttcttccttggtaggggtcattttgacaccacctttccttgcacgagggcatccggacaagcttctgtgggaagcatagtttccagtcacgtgccccgagccatcgcagcctggggttggacacttaagctcctgagagttggcagccatgagggattttagagtcttatctgctaaaggacatccagaaacactgcgatgagatgcatagtttcctgtcacgtggccacttccatcacatcctggtgttggacaggtgattagttcctttttgagatctcttgcatgaagcttgggtttagggcttggtatagaggcctctccaggaaactttttttcctctaaattttctagagagctcactgggtctttctctttctcctcctctgtcttcccgtgagttttgctatagttgataggagtgtcccagccctcttggtcacaaagagcctgatagaatgctgcattgaccagaatgctgcttgttttgaatggggaagaggaaggagttggaatagaagtgttagaggaagttaggggtgcagacttgtccaggattcgattttttttcatgcttaagtccaatgtgccattttcatccacttctatttcggctcccttggcatgcagactctgtggcttgttggagaggatgtctgtggcttccctgcagcgggtggaaaggttcaggatggcagcagctgctgctatgtgggtgtcttcactacattgaccgtagctataagagctggcacggccagggctctgggtgtgggcgcctgcactaggcagtcgattaggaaatttcactggatttggaaaatgctttgattcaggaaatggtggtgtttttcgtccttgcactgtttgtatgagagggcgtttaccgaaaacttgggcatcaaaactggcataatcaaatggtacttttccaaacttctcttgttcttttgacactgtggctctgggagaggtgatggcttgtgacgggaaattgaattcaatttgcttcaccaaacttgtcctgtgggcctggtcaggacactgcccagtttggggagaatcaagctgatttttatcctgggacattgccaatttttcagctgcagcaattggacaaccagaaagactcctgtgggtgttgcggttgctgttcacatgaccccttcctgtgcatcccggcgtgggacacttgagcacattttcatgcatggcaagaatttccaggggaacccgcactttgtgggggcaccccgaaaggctgcggtggtgcgggtagagccctgtcacgtgtcccgtgccatcacatccagggatcgggcacttggtctccctcttttcaggccttggtgaatgtttattgttaaagatttgtcttccacccatgtcgataactttggtttgcctcctttcccctgctaggtgctccagcaggaacctatccagctctttgtaggtgttatggaaaacacaacctcgctcagcctgcagagcaattgcctgctccagcaaacttaaattccccttggccttttccaggtcactaccctcttccgtcattactgccaggctctcgctatcttcctcctcaacgtcagggaatgagggctgggcattgccatccaggggttctgcgagagcattctgcgggtctttcctttctgtttcagaatcacacctgttctcacaagggataaatttgtcaccttcagtttttatttcaggaacttccaataggtcttttttatgatctgttaaaacatactttgggactctaggtggtttggtttcttctgagaagttggagccactgtcccagccattttctgcactttcagagttactttcattgtcatcagaggagcagaagggtggctgagaatcatcaatcttgtctcttccatcatcagaatgaatcagaaagcactcgtctgcttcatcgctctctgcttttaaagactggatgccactgtcatttaaattttcacttacagtctgaacagatacatttttttcaaatttccccaagtgcattaaagacttgaccatgagctcttgataacaagagtatctgtcttccttcctactggagttttcttgtgcagttgaaagaagactttcatccataggttttatcatgatttcctctgcggtagagtgaccatgtgtttccaaggggccatcgtcctctgtcctgtcactgcggtcttcttggcagtctgcttttgggctgtagtgtcggggcttcattagcagggatttccttttgttgactggaacccccaaagcctgatcttcagctgttctcttctttgccatggagcaatcataggcaacactgagctcctggattagtgaatccattggcacctcggttcctttagagcgagtacgcagcgttttatcttcagcctctgcatccatctataaacagatgtataaagtgatttcctagtacttgtacttgacgtcttttcttactggagcttacatcaggggcaataagcaggtctcttccacatcgccccagtgcacagatctggtaccttcttttaggctgaagaggaagtcctggaattgctctctttttctccaggtaacttgtatgtcaactcagtttgccctgctgtgtcagggggactaaataaatgactttgtcttatttagtgataaatcctgaaattcattctttcttgcagaaaatttctaccgtcctgccttctctaccctttgcagtatatcaaagtgctcagctttttaatcatagatttctgtgtttcttgtaggatttgaccagacattaaatagatgcttcttcaacttaagtcagcaactgtagttcctggggaaaaatggagataaaactctcaagtgatagagcagattactgcacatgatgtaagaattgaaaagtagcacaggagcttgggaattcttagtttgcgtttgattgcaactaaaaaaaaaaaaacggctttctctccaaatgtttttggcctattctattgcgccctcagttcagaaagagttctgaagctttccacctgcctattcccctttgtttgccatacactaacctaaaacaaaagatcctggaaaacagtcacactggcaaacaaagctctttctaaatcctgaaagtaa

SEQ ID NO: 18676 - RNA, 4953 nt, Homo sapiens
  source 1..4953: mol_type = other RNA
tgagtgtgtgtgtgtgagtgtgtgtgtatattttgtagcatttgaagttttgtggcaagatttctatcaaattgaatgttgtcttgtttcctatggtgggtgagacccaaggtgccagtgtttgaagtaatcattcagattggagtagcattttttcatgtgttactatattttccattcctttccagtcaacccagtaagataaatgctatttcaggggatatggtatctacaaaatttttcatttggatgtgtttgtatttgctaagtacaaatctacaccaatattgtcacttgtatattgtaccaacatatggcaggaaagcctggctggtcacaccaagtcttatttttcatcttgggatacgagttgccaacgatctgatatgacttgaaaaacaaacagacaaatctgcatcactaaaaaggcttatgtttctttaaaacatttcaaataaataattcatattaacgaaaaccgtccagccaagtcgaatactttgctgattgctatatttaattattgctaacaaattctgagcaggctgttttccagcatcctgtgcttttgtgagtgcggattccccactagtgggcgccatttgtcttcttattccttccgtgcagctcaccttaccgcaaattcatttataaatacaaaaatcagtgaaaggtgggggaagaagtgtgcaataaaaatcaaactcaactatagtgcagtccttagacaaggatttccttcaccctttcctgtttcctcattaaaacccagcaagaaagatgacttgagaatagcatttctatttaaatcctattggaaaataaattaataaacacacttgtaaaaatacggcagacttcaaaatgcagttaaaagataaaaaactctttgattagtaataaataaattataaaaatgtcacatttattttacatatactttacaaaaaaaaaaagagtacaatgaagaaataaaagaaaaacatatgaaaataaataagatctaataattgactgcattgcttttaatccaagaagtctatcatagtttttctttcctttttatatcagctggggaaaataaaattagtgcaatgttgcaaattgtaaatgcagtacggcaacctccacgccttagcagtacatgaacctctaacagatccatctggagtttactgctgttggtaacttctgttgcccggcagcgctgtgatcctacacatggatacccttcactgcctgtttgatactttccagtagagctttgcattccggggaatagtcccgttccagattgctgtacatatctgtgagtgtatttacatatgcttcaaaattctgctcactgataggtcccatctgtggaagctggatgtcagcaaggcttgaaatgagagcttggcttagacctgccagctctttcagcagactttcattgttctgttctatgagtttgttctcctcctctatcgtctttaagttgctctccatagatgtgatctgggtctgaagtttcatcatatctgcttcaattttaaggttggattcattcagttcctttatttcttcatccaaatgcctaatttcttcatcactctctattcccccagttgctttgagcttgatggtcatgagttcttcagaaaccttgccctttttgataacttgtgcattgagaggacatccagataagcttcggtgggtgacaaaaacattatttacatggcccagcccattgcagcctggcaagggacaatgtggtagctcttgtttgttcagtttccaggagagggaggctccattgagaggattctccttctgtctcttggcagccagaggacagccagaagctgtgcggtgtgatgtgtatttacctgatatgtgaccttggccatcacaccctatcacaggacatttcagttcagggtcttctttttcttccttggtaggggtcattttgacaccacctttccttgcacgagggcatccggacaagcttctgtgggaagcatagtttccagtcacgtgccccgagccatcgcagcctggggttggacacttaagctcctgagagttggcagccatgagggattttagagtcttatctgctaaaggacatccagaaacactgcgatgagatgcatagtttcctgtcacgtggccacttccatcacatcctggtgttggacaggtgattagttcctttttgagatctcttgcatgaagcttgggtttagggcttggtatagaggcctctccaggaaactttttttcctctaaattttctagagagctcactgggtctttctctttctcctcctctgtcttcccgtgagttttgctatagttgataggagtgtcccagccctcttggtcacaaagagcctgatagaatgctgcattgaccagaatgctgcttgttttgaatggggaagaggaaggagttggaatagaagtgttagaggaagttaggggtgcagacttgtccaggattcgattttttttcatgcttaagtccaatgtgccattttcatccacttctatttcggctcccttggcatgcagactctgtggcttgttggagaggatgtctgtggcttccctgcagcgggtggaaaggttcaggatggcagcagctgctgctatgtgggtgtcttcactacattgaccgtagctataagagctggcacggccagggctctgggtgtgggcgcctgcactaggcagtcgattaggaaatttcactggatttggaaaatgctttgattcaggaaatggtggtgtttttcgtccttgcactgtttgtatgagagggcgtttaccgaaaacttgggcatcaaaactggcataatcaaatggtacttttccaaacttctcttgttcttttgacactgtggctctgggagaggtgatggcttgtgacgggaaattgaattcaatttgcttcaccaaacttgtcctgtgggcctggtcaggacactgcccagtttggggagaatcaagctgatttttatcctgggacattgccaatttttcagctgcagcaattggacaaccagaaagactcctgtgggtgttgcggttgctgttcacatgaccccttcctgtgcatcccggcgtgggacacttgagcacattttcatgcatggcaagaatttccaggggaacccgcactttgtgggggcaccccgaaaggctgcggtggtgcgggtagagccctgtcacgtgtcccgtgccatcacatccagggatcgggcacttggtctccctcttttcaggccttggtgaatgtttattgttaaagatttgtcttccacccatgtcgataactttggtttgcctcctttcccctgctaggtgctccagcaggaacctatccagctctttgtaggtgttatggaaaacacaacctcgctcagcctgcagagcaattgcctgctccagcaaacttaaattccccttggccttttccaggtcactaccctcttccgtcattactgccaggctctcgctatcttcctcctcaacgtcagggaatgagggctgggcattgccatccaggggttctgcgagagcattctgcgggtctttcctttctgtttcagaatcacacctgttctcacaagggataaatttgtcaccttcagtttttatttcaggaacttccaataggtcttttttatgatctgttaaaacatactttgggactctaggtggtttggtttcttctgagaagttggagccactgtcccagccattttctgcactttcagagttactttcattgtcatcagaggagcagaagggtggctgagaatcatcaatcttgtctcttccatcatcagaatgaatcagaaagcactcgtctgcttcatcgctctctgcttttaaagactggatgccactgtcatttaaattttcacttacagtctgaacagatacatttttttcaaatttccccaagtgcattaaagacttgaccatgagctcttgataacaagagtatctgtcttccttcctactggagttttcttgtgcagttgaaagaagactttcatccataggttttatcatgatttcctctgcggtagagtgaccatgtgtttccaaggggccatcgtcctctgtcctgtcactgcggtcttcttggcagtctgcttttgggctgtagtgtcggggcttcattagcagggatttccttttgttgactggaacccccaaagcctgatcttcagctgttctcttctttgccatggagcaatcataggcaacactgagctcctggattagtgaatccattggcacctcggttcctttagagcgagtacgcagcgttttatcttcagcctctgcatccatctataaacagatgtataaagtgatttcctagtacttgtacttgacgtcttttcttactggagcttacatcaggggcaataagcaggtctcttccacatcgccccagtgcacagatctggtaccttcttttaggctgaagaggaagtcctggaattgctctctttttctccaggtaacttgtatgtcaactcagtttgccctgctgtgtcagggggactaaataaatgactttgtcttatttagtgataaatcctgaaattcattctttcttgcagaaaatttctaccgtcctgccttctctaccctttgcagtatatcaaagtgctcagctttttaatcatagatttctgtgtttcttgtaggatttgaccagacattaaatagatgcttcttcaacttaagtcagcaactgtagttccttccctaaaagctactggatctgaactggagagtttccatcactccggtgcctcctagcctttgttctgcctctcacgctgacatcagggaagcagtgatgtagaataaagcaggggtgggctaggttagtccagtgtttgtgtcgttgtgtggtgtgcagggacactctgtgat

SEQ ID NO: 18677 - RNA, 5032 nt, Homo sapiens
  source 1..5032: mol_type = other RNA
tgagtgtgtgtgtgtgagtgtgtgtgtatattttgtagcatttgaagttttgtggcaagatttctatcaaattgaatgttgtcttgtttcctatggtgggtgagacccaaggtgccagtgtttgaagtaatcattcagattggagtagcattttttcatgtgttactatattttccattcctttccagtcaacccagtaagataaatgctatttcaggggatatggtatctacaaaatttttcatttggatgtgtttgtatttgctaagtacaaatctacaccaatattgtcacttgtatattgtaccaacatatggcaggaaagcctggctggtcacaccaagtcttatttttcatcttgggatacgagttgccaacgatctgatatgacttgaaaaacaaacagacaaatctgcatcactaaaaaggcttatgtttctttaaaacatttcaaataaataattcatattaacgaaaaccgtccagccaagtcgaatactttgctgattgctatatttaattattgctaacaaattctgagcaggctgttttccagcatcctgtgcttttgtgagtgcggattccccactagtgggcgccatttgtcttcttattccttccgtgcagctcaccttaccgcaaattcatttataaatacaaaaatcagtgaaaggtgggggaagaagtgtgcaataaaaatcaaactcaactatagtgcagtccttagacaaggatttccttcaccctttcctgtttcctcattaaaacccagcaagaaagatgacttgagaatagcatttctatttaaatcctattggaaaataaattaataaacacacttgtaaaaatacggcagacttcaaaatgcagttaaaagataaaaaactctttgattagtaataaataaattataaaaatgtcacatttattttacatatactttacaaaaaaaaaaagagtacaatgaagaaataaaagaaaaacatatgaaaataaataagatctaataattgactgcattgcttttaatccaagaagtctatcatagtttttctttcctttttatatcagctggggaaaataaaattagtgcaatgttgcaaattgtaaatgcagtacggcaacctccacgccttagcagtacatgaacctctaacagatccatctggagtttactgctgttggtaacttctgttgcccggcagcgctgtgatcctacacatggatacccttcactgcctgtttgatactttccagtagagctttgcattccggggaatagtcccgttccagattgctgtacatatctgtgagtgtatttacatatgcttcaaaattctgctcactgataggtcccatctgtggaagctggatgtcagcaaggcttgaaatgagagcttggcttagacctgccagctctttcagcagactttcattgttctgttctatgagtttgttctcctcctctatcgtctttaagttgctctccatagatgtgatctgggtctgaagtttcatcatatctgcttcaattttaaggttggattcattcagttcctttatttcttcatccaaatgcctaatttcttcatcactctctattcccccagttgctttgagcttgatggtcatgagttcttcagaaaccttgccctttttgataacttgtgcattgagaggacatccagataagcttcggtgggtgacaaaaacattatttacatggcccagcccattgcagcctggcaagggacaatgtggtagctcttgtttgttcagtttccaggagagggaggctccattgagaggattctccttctgtctcttggcagccagaggacagccagaagctgtgcggtgtgatgtgtatttacctgatatgtgaccttggccatcacaccctatcacaggacatttcagttcagggtcttctttttcttccttggtaggggtcattttgacaccacctttccttgcacgagggcatccggacaagcttctgtgggaagcatagtttccagtcacgtgccccgagccatcgcagcctggggttggacacttaagctcctgagagttggcagccatgagggattttagagtcttatctgctaaaggacatccagaaacactgcgatgagatgcatagtttcctgtcacgtggccacttccatcacatcctggtgttggacaggtgattagttcctttttgagatctcttgcatgaagcttgggtttagggcttggtatagaggcctctccaggaaactttttttcctctaaattttctagagagctcactgggtctttctctttctcctcctctgtcttcccgtgagttttgctatagttgataggagtgtcccagccctcttggtcacaaagagcctgatagaatgctgcattgaccagaatgctgcttgttttgaatggggaagaggaaggagttggaatagaagtgttagaggaagttaggggtgcagacttgtccaggattcgattttttttcatgcttaagtccaatgtgccattttcatccacttctatttcggctcccttggcatgcagactctgtggcttgttggagaggatgtctgtggcttccctgcagcgggtggaaaggttcaggatggcagcagctgctgctatgtgggtgtcttcactacattgaccgtagctataagagctggcacggccagggctctgggtgtgggcgcctgcactaggcagtcgattaggaaatttcactggatttggaaaatgctttgattcaggaaatggtggtgtttttcgtccttgcactgtttgtatgagagggcgtttaccgaaaacttgggcatcaaaactggcataatcaaatggtacttttccaaacttctcttgttcttttgacactgtggctctgggagaggtgatggcttgtgacgggaaattgaattcaatttgcttcaccaaacttgtcctgtgggcctggtcaggacactgcccagtttggggagaatcaagctgatttttatcctgggacattgccaatttttcagctgcagcaattggacaaccagaaagactcctgtgggtgttgcggttgctgttcacatgaccccttcctgtgcatcccggcgtgggacacttgagcacattttcatgcatggcaagaatttccaggggaacccgcactttgtgggggcaccccgaaaggctgcggtggtgcgggtagagccctgtcacgtgtcccgtgccatcacatccagggatcgggcacttggtctccctcttttcaggccttggtgaatgtttattgttaaagatttgtcttccacccatgtcgataactttggtttgcctcctttcccctgctaggtgctccagcaggaacctatccagctctttgtaggtgttatggaaaacacaacctcgctcagcctgcagagcaattgcctgctccagcaaacttaaattccccttggccttttccaggtcactaccctcttccgtcattactgccaggctctcgctatcttcctcctcaacgtcagggaatgagggctgggcattgccatccaggggttctgcgagagcattctgcgggtctttcctttctgtttcagaatcacacctgttctcacaagggataaatttgtcaccttcagtttttatttcaggaacttccaataggtcttttttatgatctgttaaaacatactttgggactctaggtggtttggtttcttctgagaagttggagccactgtcccagccattttctgcactttcagagttactttcattgtcatcagaggagcagaagggtggctgagaatcatcaatcttgtctcttccatcatcagaatgaatcagaaagcactcgtctgcttcatcgctctctgcttttaaagactggatgccactgtcatttaaattttcacttacagtctgaacagatacatttttttcaaatttccccaagtgcattaaagacttgaccatgagctcttgataacaagagtatctgtcttccttcctactggagttttcttgtgcagttgaaagaagactttcatccataggttttatcatgatttcctctgcggtagagtgaccatgtgtttccaaggggccatcgtcctctgtcctgtcactgcggtcttcttggcagtctgcttttgggctgtagtgtcggggcttcattagcagggatttccttttgttgactggaacccccaaagcctgatcttcagctgttctcttctttgccatggagcaatcataggcaacactgagctcctggattagtgaatccattggcacctcggttcctttagagcgagtacgcagcgttttatcttcagcctctgcatccatctataaacagatgtataaagtgatttcctagtacttgtacttgacgtcttttcttactggagcttacatcaggggcaataagcaggtctcttccacatcgccccagtgcacagatctggtaccttcttttaggctgaagaggaagtcctggaattgctctctttttctccaggtaacttgtatgtcaactcagtttgccctgctgtgtcagggggactaaataaatgactttgtcttatttagtgataaatcctgaaattcattctttcttgcagaaaatttctaccgtcctgccttctctaccctttgcagtatatcaaagtgctcagctttttaatcatagatttctgtgtttcttgtaggatttgaccagacattaaatagatgcttcttcaacttaagtcagcaactgtagttccttccctaaaagctactggatctgaactggagagtttccatcactccttagtcttgatatgagcacgcagacacataaaatggaattgtcacaatgcttcagggacactcacaaaattgggggctcggtgcctcctagcctttgttctgcctctcacgctgacatcagggaagcagtgatgtagaataaagcaggggtgggctaggttagtccagtgtttgtgtcgttgtgtggtgtgcagggacactctgtgat

SEQ ID NO: 18678 - RNA, 5068 nt, Homo sapiens
  source 1..5068: mol_type = other RNA
tgagtgtgtgtgtgtgagtgtgtgtgtatattttgtagcatttgaagttttgtggcaagatttctatcaaattgaatgttgtcttgtttcctatggtgggtgagacccaaggtgccagtgtttgaagtaatcattcagattggagtagcattttttcatgtgttactatattttccattcctttccagtcaacccagtaagataaatgctatttcaggggatatggtatctacaaaatttttcatttggatgtgtttgtatttgctaagtacaaatctacaccaatattgtcacttgtatattgtaccaacatatggcaggaaagcctggctggtcacaccaagtcttatttttcatcttgggatacgagttgccaacgatctgatatgacttgaaaaacaaacagacaaatctgcatcactaaaaaggcttatgtttctttaaaacatttcaaataaataattcatattaacgaaaaccgtccagccaagtcgaatactttgctgattgctatatttaattattgctaacaaattctgagcaggctgttttccagcatcctgtgcttttgtgagtgcggattccccactagtgggcgccatttgtcttcttattccttccgtgcagctcaccttaccgcaaattcatttataaatacaaaaatcagtgaaaggtgggggaagaagtgtgcaataaaaatcaaactcaactatagtgcagtccttagacaaggatttccttcaccctttcctgtttcctcattaaaacccagcaagaaagatgacttgagaatagcatttctatttaaatcctattggaaaataaattaataaacacacttgtaaaaatacggcagacttcaaaatgcagttaaaagataaaaaactctttgattagtaataaataaattataaaaatgtcacatttattttacatatactttacaaaaaaaaaaagagtacaatgaagaaataaaagaaaaacatatgaaaataaataagatctaataattgactgcattgcttttaatccaagaagtctatcatagtttttctttcctttttatatcagctggggaaaataaaattagtgcaatgttgcaaattgtaaatgcagtacggcaacctccacgccttagcagtacatgaacctctaacagatccatctggagtttactgctgttggtaacttctgttgcccggcagcgctgtgatcctacacatggatacccttcactgcctgtttgatactttccagtagagctttgcattccggggaatagtcccgttccagattgctgtacatatctgtgagtgtatttacatatgcttcaaaattctgctcactgataggtcccatctgtggaagctggatgtcagcaaggcttgaaatgagagcttggcttagacctgccagctctttcagcagactttcattgttctgttctatgagtttgttctcctcctctatcgtctttaagttgctctccatagatgtgatctgggtctgaagtttcatcatatctgcttcaattttaaggttggattcattcagttcctttatttcttcatccaaatgcctaatttcttcatcactctctattcccccagttgctttgagcttgatggtcatgagttcttcagaaaccttgccctttttgataacttgtgcattgagaggacatccagataagcttcggtgggtgacaaaaacattatttacatggcccagcccattgcagcctggcaagggacaatgtggtagctcttgtttgttcagtttccaggagagggaggctccattgagaggattctccttctgtctcttggcagccagaggacagccagaagctgtgcggtgtgatgtgtatttacctgatatgtgaccttggccatcacaccctatcacaggacatttcagttcagggtcttctttttcttccttggtaggggtcattttgacaccacctttccttgcacgagggcatccggacaagcttctgtgggaagcatagtttccagtcacgtgccccgagccatcgcagcctggggttggacacttaagctcctgagagttggcagccatgagggattttagagtcttatctgctaaaggacatccagaaacactgcgatgagatgcatagtttcctgtcacgtggccacttccatcacatcctggtgttggacaggtgattagttcctttttgagatctcttgcatgaagcttgggtttagggcttggtatagaggcctctccaggaaactttttttcctctaaattttctagagagctcactgggtctttctctttctcctcctctgtcttcccgtgagttttgctatagttgataggagtgtcccagccctcttggtcacaaagagcctgatagaatgctgcattgaccagaatgctgcttgttttgaatggggaagaggaaggagttggaatagaagtgttagaggaagttaggggtgcagacttgtccaggattcgattttttttcatgcttaagtccaatgtgccattttcatccacttctatttcggctcccttggcatgcagactctgtggcttgttggagaggatgtctgtggcttccctgcagcgggtggaaaggttcaggatggcagcagctgctgctatgtgggtgtcttcactacattgaccgtagctataagagctggcacggccagggctctgggtgtgggcgcctgcactaggcagtcgattaggaaatttcactggatttggaaaatgctttgattcaggaaatggtggtgtttttcgtccttgcactgtttgtatgagagggcgtttaccgaaaacttgggcatcaaaactggcataatcaaatggtacttttccaaacttctcttgttcttttgacactgtggctctgggagaggtgatggcttgtgacgggaaattgaattcaatttgcttcaccaaacttgtcctgtgggcctggtcaggacactgcccagtttggggagaatcaagctgatttttatcctgggacattgccaatttttcagctgcagcaattggacaaccagaaagactcctgtgggtgttgcggttgctgttcacatgaccccttcctgtgcatcccggcgtgggacacttgagcacattttcatgcatggcaagaatttccaggggaacccgcactttgtgggggcaccccgaaaggctgcggtggtgcgggtagagccctgtcacgtgtcccgtgccatcacatccagggatcgggcacttggtctccctcttttcaggccttggtgaatgtttattgttaaagatttgtcttccacccatgtcgataactttggtttgcctcctttcccctgctaggtgctccagcaggaacctatccagctctttgtaggtgttatggaaaacacaacctcgctcagcctgcagagcaattgcctgctccagcaaacttaaattccccttggccttttccaggtcactaccctcttccgtcattactgccaggctctcgctatcttcctcctcaacgtcagggaatgagggctgggcattgccatccaggggttctgcgagagcattctgcgggtctttcctttctgtttcagaatcacacctgttctcacaagggataaatttgtcaccttcagtttttatttcaggaacttccaataggtcttttttatgatctgttaaaacatactttgggactctaggtggtttggtttcttctgagaagttggagccactgtcccagccattttctgcactttcagagttactttcattgtcatcagaggagcagaagggtggctgagaatcatcaatcttgtctcttccatcatcagaatgaatcagaaagcactcgtctgcttcatcgctctctgcttttaaagactggatgccactgtcatttaaattttcacttacagtctgaacagatacatttttttcaaatttccccaagtgcattaaagacttgaccatgagctcttgataacaagagtatctgtcttccttcctactggagttttcttgtgcagttgaaagaagactttcatccataggttttatcatgatttcctctgcggtagagtgaccatgtgtttccaaggggccatcgtcctctgtcctgtcactgcggtcttcttggcagtctgcttttgggctgtagtgtcggggcttcattagcagggatttccttttgttgactggaacccccaaagcctgatcttcagctgttctcttctttgccatggagcaatcataggcaacactgagctcctggattagtgaatccattggcacctcggttcctttagagcgagtacgcagcgttttatcttcagcctctgcatccatctataaacagatgtataaagtgatttcctagtacttgtacttgacgtcttttcttactggagcttacatcaggggcaataagcaggtctcttccacatcgccccagtgcacagatctggtaccttcttttaggctgaagaggaagtcctggaattgctctctttttctccaggtaacttgtatgtcaactcagtttgccctgctgtgtcagggggactaaataaatgactttgtcttatttagtgataaatcctgaaattcattctttcttgcagaaaatttctaccgtcctgccttctctaccctttgcagtatatcaaagtgctcagctttttaatcatagatttctgtgtttcttgtaggatttgaccagacattaaatagatgcttcttcaacttaagtcagcaactgtagttccttccctaaaagctactggatctgaactggagagtttccatcactccttagtcttgatatgagcacgcagacacataaaatggaattgtcacaatgcttcagggacactcacaaaattgggggctctgaatgtcttgtaacaatatcatcctctcttgaactaaacatcctctgaatacacaaatctaaggcagacagacatttcagcaaggcaaataagactttctggcaacttcctgttgccatatttctctcaaaggatcctgcaatgttacacttcaatcctgcaaa

SEQ ID NO: 18679 - RNA, 5102 nt, Homo sapiens
  source 1..5102: mol_type = other RNA
tgagtgtgtgtgtgtgagtgtgtgtgtatattttgtagcatttgaagttttgtggcaagatttctatcaaattgaatgttgtcttgtttcctatggtgggtgagacccaaggtgccagtgtttgaagtaatcattcagattggagtagcattttttcatgtgttactatattttccattcctttccagtcaacccagtaagataaatgctatttcaggggatatggtatctacaaaatttttcatttggatgtgtttgtatttgctaagtacaaatctacaccaatattgtcacttgtatattgtaccaacatatggcaggaaagcctggctggtcacaccaagtcttatttttcatcttgggatacgagttgccaacgatctgatatgacttgaaaaacaaacagacaaatctgcatcactaaaaaggcttatgtttctttaaaacatttcaaataaataattcatattaacgaaaaccgtccagccaagtcgaatactttgctgattgctatatttaattattgctaacaaattctgagcaggctgttttccagcatcctgtgcttttgtgagtgcggattccccactagtgggcgccatttgtcttcttattccttccgtgcagctcaccttaccgcaaattcatttataaatacaaaaatcagtgaaaggtgggggaagaagtgtgcaataaaaatcaaactcaactatagtgcagtccttagacaaggatttccttcaccctttcctgtttcctcattaaaacccagcaagaaagatgacttgagaatagcatttctatttaaatcctattggaaaataaattaataaacacacttgtaaaaatacggcagacttcaaaatgcagttaaaagataaaaaactctttgattagtaataaataaattataaaaatgtcacatttattttacatatactttacaaaaaaaaaaagagtacaatgaagaaataaaagaaaaacatatgaaaataaataagatctaataattgactgcattgcttttaatccaagaagtctatcatagtttttctttcctttttatatcagctggggaaaataaaattagtgcaatgttgcaaattgtaaatgcagtacggcaacctccacgccttagcagtacatgaacctctaacagatccatctggagtttactgctgttggtaacttctgttgcccggcagcgctgtgatcctacacatggatacccttcactgcctgtttgatactttccagtagagctttgcattccggggaatagtcccgttccagattgctgtacatatctgtgagtgtatttacatatgcttcaaaattctgctcactgataggtcccatctgtggaagctggatgtcagcaaggcttgaaatgagagcttggcttagacctgccagctctttcagcagactttcattgttctgttctatgagtttgttctcctcctctatcgtctttaagttgctctccatagatgtgatctgggtctgaagtttcatcatatctgcttcaattttaaggttggattcattcagttcctttatttcttcatccaaatgcctaatttcttcatcactctctattcccccagttgctttgagcttgatggtcatgagttcttcagaaaccttgccctttttgataacttgtgcattgagaggacatccagataagcttcggtgggtgacaaaaacattatttacatggcccagcccattgcagcctggcaagggacaatgtggtagctcttgtttgttcagtttccaggagagggaggctccattgagaggattctccttctgtctcttggcagccagaggacagccagaagctgtgcggtgtgatgtgtatttacctgatatgtgaccttggccatcacaccctatcacaggacatttcagttcagggtcttctttttcttccttggtaggggtcattttgacaccacctttccttgcacgagggcatccggacaagcttctgtgggaagcatagtttccagtcacgtgccccgagccatcgcagcctggggttggacacttaagctcctgagagttggcagccatgagggattttagagtcttatctgctaaaggacatccagaaacactgcgatgagatgcatagtttcctgtcacgtggccacttccatcacatcctggtgttggacaggtgattagttcctttttgagatctcttgcatgaagcttgggtttagggcttggtatagaggcctctccaggaaactttttttcctctaaattttctagagagctcactgggtctttctctttctcctcctctgtcttcccgtgagttttgctatagttgataggagtgtcccagccctcttggtcacaaagagcctgatagaatgctgcattgaccagaatgctgcttgttttgaatggggaagaggaaggagttggaatagaagtgttagaggaagttaggggtgcagacttgtccaggattcgattttttttcatgcttaagtccaatgtgccattttcatccacttctatttcggctcccttggcatgcagactctgtggcttgttggagaggatgtctgtggcttccctgcagcgggtggaaaggttcaggatggcagcagctgctgctatgtgggtgtcttcactacattgaccgtagctataagagctggcacggccagggctctgggtgtgggcgcctgcactaggcagtcgattaggaaatttcactggatttggaaaatgctttgattcaggaaatggtggtgtttttcgtccttgcactgtttgtatgagagggcgtttaccgaaaacttgggcatcaaaactggcataatcaaatggtacttttccaaacttctcttgttcttttgacactgtggctctgggagaggtgatggcttgtgacgggaaattgaattcaatttgcttcaccaaacttgtcctgtgggcctggtcaggacactgcccagtttggggagaatcaagctgatttttatcctgggacattgccaatttttcagctgcagcaattggacaaccagaaagactcctgtgggtgttgcggttgctgttcacatgaccccttcctgtgcatcccggcgtgggacacttgagcacattttcatgcatggcaagaatttccaggggaacccgcactttgtgggggcaccccgaaaggctgcggtggtgcgggtagagccctgtcacgtgtcccgtgccatcacatccagggatcgggcacttggtctccctcttttcaggccttggtgaatgtttattgttaaagatttgtcttccacccatgtcgataactttggtttgcctcctttcccctgctaggtgctccagcaggaacctatccagctctttgtaggtgttatggaaaacacaacctcgctcagcctgcagagcaattgcctgctccagcaaacttaaattccccttggccttttccaggtcactaccctcttccgtcattactgccaggctctcgctatcttcctcctcaacgtcagggaatgagggctgggcattgccatccaggggttctgcgagagcattctgcgggtctttcctttctgtttcagaatcacacctgttctcacaagggataaatttgtcaccttcagtttttatttcaggaacttccaataggtcttttttatgatctgttaaaacatactttgggactctaggtggtttggtttcttctgagaagttggagccactgtcccagccattttctgcactttcagagttactttcattgtcatcagaggagcagaagggtggctgagaatcatcaatcttgtctcttccatcatcagaatgaatcagaaagcactcgtctgcttcatcgctctctgcttttaaagactggatgccactgtcatttaaattttcacttacagtctgaacagatacatttttttcaaatttccccaagtgcattaaagacttgaccatgagctcttgataacaagagtatctgtcttccttcctactggagttttcttgtgcagttgaaagaagactttcatccataggttttatcatgatttcctctgcggtagagtgaccatgtgtttccaaggggccatcgtcctctgtcctgtcactgcggtcttcttggcagtctgcttttgggctgtagtgtcggggcttcattagcagggatttccttttgttgactggaacccccaaagcctgatcttcagctgttctcttctttgccatggagcaatcataggcaacactgagctcctggattagtgaatccattggcacctcggttcctttagagcgagtacgcagcgttttatcttcagcctctgcatccatctataaacagatgtataaagtgatttcctagtacttgtacttgacgtcttttcttactggagcttacatcaggggcaataagcaggtctcttccacatcgccccagtgcacagatctggtaccttcttttaggctgaagaggaagtcctggaattgctctctttttctccaggtaacttgtatgtcaactcagtttgccctgctgtgtcagggggactaaataaatgactttgtcttatttagtgataaatcctgaaattcattctttcttgcagaaaatttctaccgtcctgccttctctaccctttgcagtatatcaaagtgctcagctttttaatcatagatttctgtgtttcttgtaggatttgaccagacattaaatagatgcttcttcaacttaagtcagcaactgtagttccttccctaaaagctactggatctgaactggagagtttccatcactccttagtcttgatatgagcacgcagacacataaaatggaattgtcacaatgcttcagggacactcacaaaattgggggctctttacctggcgaacgtctacaggtgtgtcgaaagttatcttttcctggatgtgttccaaaatgctcttatgctatttctcttaggatttctccacgctgccccattcagaaattttattattttctctagtattcccctgaggtcacattcagttaaaaacatcctgcccttctccctacaaaaaggttccatagaatc

SEQ ID NO: 18680 - RNA, 5001 nt, Homo sapiens
  source 1..5001: mol_type = other RNA
tgagtgtgtgtgtgtgagtgtgtgtgtatattttgtagcatttgaagttttgtggcaagatttctatcaaattgaatgttgtcttgtttcctatggtgggtgagacccaaggtgccagtgtttgaagtaatcattcagattggagtagcattttttcatgtgttactatattttccattcctttccagtcaacccagtaagataaatgctatttcaggggatatggtatctacaaaatttttcatttggatgtgtttgtatttgctaagtacaaatctacaccaatattgtcacttgtatattgtaccaacatatggcaggaaagcctggctggtcacaccaagtcttatttttcatcttgggatacgagttgccaacgatctgatatgacttgaaaaacaaacagacaaatctgcatcactaaaaaggcttatgtttctttaaaacatttcaaataaataattcatattaacgaaaaccgtccagccaagtcgaatactttgctgattgctatatttaattattgctaacaaattctgagcaggctgttttccagcatcctgtgcttttgtgagtgcggattccccactagtgggcgccatttgtcttcttattccttccgtgcagctcaccttaccgcaaattcatttataaatacaaaaatcagtgaaaggtgggggaagaagtgtgcaataaaaatcaaactcaactatagtgcagtccttagacaaggatttccttcaccctttcctgtttcctcattaaaacccagcaagaaagatgacttgagaatagcatttctatttaaatcctattggaaaataaattaataaacacacttgtaaaaatacggcagacttcaaaatgcagttaaaagataaaaaactctttgattagtaataaataaattataaaaatgtcacatttattttacatatactttacaaaaaaaaaaagagtacaatgaagaaataaaagaaaaacatatgaaaataaataagatctaataattgactgcattgcttttaatccaagaagtctatcatagtttttctttcctttttatatcagctggggaaaataaaattagtgcaatgttgcaaattgtaaatgcagtacggcaacctccacgccttagcagtacatgaacctctaacagatccatctggagtttactgctgttggtaacttctgttgcccggcagcgctgtgatcctacacatggatacccttcactgcctgtttgatactttccagtagagctttgcattccggggaatagtcccgttccagattgctgtacatatctgtgagtgtatttacatatgcttcaaaattctgctcactgataggtcccatctgtggaagctggatgtcagcaaggcttgaaatgagagcttggcttagacctgccagctctttcagcagactttcattgttctgttctatgagtttgttctcctcctctatcgtctttaagttgctctccatagatgtgatctgggtctgaagtttcatcatatctgcttcaattttaaggttggattcattcagttcctttatttcttcatccaaatgcctaatttcttcatcactctctattcccccagttgctttgagcttgatggtcatgagttcttcagaaaccttgccctttttgataacttgtgcattgagaggacatccagataagcttcggtgggtgacaaaaacattatttacatggcccagcccattgcagcctggcaagggacaatgtggtagctcttgtttgttcagtttccaggagagggaggctccattgagaggattctccttctgtctcttggcagccagaggacagccagaagctgtgcggtgtgatgtgtatttacctgatatgtgaccttggccatcacaccctatcacaggacatttcagttcagggtcttctttttcttccttggtaggggtcattttgacaccacctttccttgcacgagggcatccggacaagcttctgtgggaagcatagtttccagtcacgtgccccgagccatcgcagcctggggttggacacttaagctcctgagagttggcagccatgagggattttagagtcttatctgctaaaggacatccagaaacactgcgatgagatgcatagtttcctgtcacgtggccacttccatcacatcctggtgttggacaggtgattagttcctttttgagatctcttgcatgaagcttgggtttagggcttggtatagaggcctctccaggaaactttttttcctctaaattttctagagagctcactgggtctttctctttctcctcctctgtcttcccgtgagttttgctatagttgataggagtgtcccagccctcttggtcacaaagagcctgatagaatgctgcattgaccagaatgctgcttgttttgaatggggaagaggaaggagttggaatagaagtgttagaggaagttaggggtgcagacttgtccaggattcgattttttttcatgcttaagtccaatgtgccattttcatccacttctatttcggctcccttggcatgcagactctgtggcttgttggagaggatgtctgtggcttccctgcagcgggtggaaaggttcaggatggcagcagctgctgctatgtgggtgtcttcactacattgaccgtagctataagagctggcacggccagggctctgggtgtgggcgcctgcactaggcagtcgattaggaaatttcactggatttggaaaatgctttgattcaggaaatggtggtgtttttcgtccttgcactgtttgtatgagagggcgtttaccgaaaacttgggcatcaaaactggcataatcaaatggtacttttccaaacttctcttgttcttttgacactgtggctctgggagaggtgatggcttgtgacgggaaattgaattcaatttgcttcaccaaacttgtcctgtgggcctggtcaggacactgcccagtttggggagaatcaagctgatttttatcctgggacattgccaatttttcagctgcagcaattggacaaccagaaagactcctgtgggtgttgcggttgctgttcacatgaccccttcctgtgcatcccggcgtgggacacttgagcacattttcatgcatggcaagaatttccaggggaacccgcactttgtgggggcaccccgaaaggctgcggtggtgcgggtagagccctgtcacgtgtcccgtgccatcacatccagggatcgggcacttggtctccctcttttcaggccttggtgaatgtttattgttaaagatttgtcttccacccatgtcgataactttggtttgcctcctttcccctgctaggtgctccagcaggaacctatccagctctttgtaggtgttatggaaaacacaacctcgctcagcctgcagagcaattgcctgctccagcaaacttaaattccccttggccttttccaggtcactaccctcttccgtcattactgccaggctctcgctatcttcctcctcaacgtcagggaatgagggctgggcattgccatccaggggttctgcgagagcattctgcgggtctttcctttctgtttcagaatcacacctgttctcacaagggataaatttgtcaccttcagtttttatttcaggaacttccaataggtcttttttatgatctgttaaaacatactttgggactctaggtggtttggtttcttctgagaagttggagccactgtcccagccattttctgcactttcagagttactttcattgtcatcagaggagcagaagggtggctgagaatcatcaatcttgtctcttccatcatcagaatgaatcagaaagcactcgtctgcttcatcgctctctgcttttaaagactggatgccactgtcatttaaattttcacttacagtctgaacagatacatttttttcaaatttccccaagtgcattaaagacttgaccatgagctcttgataacaagagtatctgtcttccttcctactggagttttcttgtgcagttgaaagaagactttcatccataggttttatcatgatttcctctgcggtagagtgaccatgtgtttccaaggggccatcgtcctctgtcctgtcactgcggtcttcttggcagtctgcttttgggctgtagtgtcggggcttcattagcagggatttccttttgttgactggaacccccaaagcctgatcttcagctgttctcttctttgccatggagcaatcataggcaacactgagctcctggattagtgaatccattggcacctcggttcctttagagcgagtacgcagcgttttatcttcagcctctgcatccatctataaacagatgtataaagtgatttcctagtacttgtacttgacgtcttttcttactggagcttacatcaggggcaataagcaggtctcttccacatcgccccagtgcacagatctggtaccttcttttaggctgaagaggaagtcctggaattgctctctttttctccaggtaacttgtatgtcaactcagtttgccctgctgtgtcagggggactaaataaatgactttgtcttatttagtgataaatcctgaaattcattctttcttgcagaaaatttctaccgtcctgccttctctaccctttgcagtatatcaaagtgctcagctttttaatcatagatttctgtgtttcttgtaggatttgaccagacattaaatagatgcttcttcaacttaagtcagcaactgtagttccttccctaaaagctactggatctgaactggagagtttccatcactccttagtcttgatatgagcacgcagacacataaaatggaattgtcacaatgcttcagggacactcacaaaattgggggctttttttgtttgtttccaaaacttatatttctctcctccctggtgggctgaacggaaacactaaagctgtttctttgaaaggtagttcccatgatatgac

SEQ ID NO: 18681 - RNA, 5023 nt, Homo sapiens
  source 1..5023: mol_type = other RNA
tgagtgtgtgtgtgtgagtgtgtgtgtatattttgtagcatttgaagttttgtggcaagatttctatcaaattgaatgttgtcttgtttcctatggtgggtgagacccaaggtgccagtgtttgaagtaatcattcagattggagtagcattttttcatgtgttactatattttccattcctttccagtcaacccagtaagataaatgctatttcaggggatatggtatctacaaaatttttcatttggatgtgtttgtatttgctaagtacaaatctacaccaatattgtcacttgtatattgtaccaacatatggcaggaaagcctggctggtcacaccaagtcttatttttcatcttgggatacgagttgccaacgatctgatatgacttgaaaaacaaacagacaaatctgcatcactaaaaaggcttatgtttctttaaaacatttcaaataaataattcatattaacgaaaaccgtccagccaagtcgaatactttgctgattgctatatttaattattgctaacaaattctgagcaggctgttttccagcatcctgtgcttttgtgagtgcggattccccactagtgggcgccatttgtcttcttattccttccgtgcagctcaccttaccgcaaattcatttataaatacaaaaatcagtgaaaggtgggggaagaagtgtgcaataaaaatcaaactcaactatagtgcagtccttagacaaggatttccttcaccctttcctgtttcctcattaaaacccagcaagaaagatgacttgagaatagcatttctatttaaatcctattggaaaataaattaataaacacacttgtaaaaatacggcagacttcaaaatgcagttaaaagataaaaaactctttgattagtaataaataaattataaaaatgtcacatttattttacatatactttacaaaaaaaaaaagagtacaatgaagaaataaaagaaaaacatatgaaaataaataagatctaataattgactgcattgcttttaatccaagaagtctatcatagtttttctttcctttttatatcagctggggaaaataaaattagtgcaatgttgcaaattgtaaatgcagtacggcaacctccacgccttagcagtacatgaacctctaacagatccatctggagtttactgctgttggtaacttctgttgcccggcagcgctgtgatcctacacatggatacccttcactgcctgtttgatactttccagtagagctttgcattccggggaatagtcccgttccagattgctgtacatatctgtgagtgtatttacatatgcttcaaaattctgctcactgataggtcccatctgtggaagctggatgtcagcaaggcttgaaatgagagcttggcttagacctgccagctctttcagcagactttcattgttctgttctatgagtttgttctcctcctctatcgtctttaagttgctctccatagatgtgatctgggtctgaagtttcatcatatctgcttcaattttaaggttggattcattcagttcctttatttcttcatccaaatgcctaatttcttcatcactctctattcccccagttgctttgagcttgatggtcatgagttcttcagaaaccttgccctttttgataacttgtgcattgagaggacatccagataagcttcggtgggtgacaaaaacattatttacatggcccagcccattgcagcctggcaagggacaatgtggtagctcttgtttgttcagtttccaggagagggaggctccattgagaggattctccttctgtctcttggcagccagaggacagccagaagctgtgcggtgtgatgtgtatttacctgatatgtgaccttggccatcacaccctatcacaggacatttcagttcagggtcttctttttcttccttggtaggggtcattttgacaccacctttccttgcacgagggcatccggacaagcttctgtgggaagcatagtttccagtcacgtgccccgagccatcgcagcctggggttggacacttaagctcctgagagttggcagccatgagggattttagagtcttatctgctaaaggacatccagaaacactgcgatgagatgcatagtttcctgtcacgtggccacttccatcacatcctggtgttggacaggtgattagttcctttttgagatctcttgcatgaagcttgggtttagggcttggtatagaggcctctccaggaaactttttttcctctaaattttctagagagctcactgggtctttctctttctcctcctctgtcttcccgtgagttttgctatagttgataggagtgtcccagccctcttggtcacaaagagcctgatagaatgctgcattgaccagaatgctgcttgttttgaatggggaagaggaaggagttggaatagaagtgttagaggaagttaggggtgcagacttgtccaggattcgattttttttcatgcttaagtccaatgtgccattttcatccacttctatttcggctcccttggcatgcagactctgtggcttgttggagaggatgtctgtggcttccctgcagcgggtggaaaggttcaggatggcagcagctgctgctatgtgggtgtcttcactacattgaccgtagctataagagctggcacggccagggctctgggtgtgggcgcctgcactaggcagtcgattaggaaatttcactggatttggaaaatgctttgattcaggaaatggtggtgtttttcgtccttgcactgtttgtatgagagggcgtttaccgaaaacttgggcatcaaaactggcataatcaaatggtacttttccaaacttctcttgttcttttgacactgtggctctgggagaggtgatggcttgtgacgggaaattgaattcaatttgcttcaccaaacttgtcctgtgggcctggtcaggacactgcccagtttggggagaatcaagctgatttttatcctgggacattgccaatttttcagctgcagcaattggacaaccagaaagactcctgtgggtgttgcggttgctgttcacatgaccccttcctgtgcatcccggcgtgggacacttgagcacattttcatgcatggcaagaatttccaggggaacccgcactttgtgggggcaccccgaaaggctgcggtggtgcgggtagagccctgtcacgtgtcccgtgccatcacatccagggatcgggcacttggtctccctcttttcaggccttggtgaatgtttattgttaaagatttgtcttccacccatgtcgataactttggtttgcctcctttcccctgctaggtgctccagcaggaacctatccagctctttgtaggtgttatggaaaacacaacctcgctcagcctgcagagcaattgcctgctccagcaaacttaaattccccttggccttttccaggtcactaccctcttccgtcattactgccaggctctcgctatcttcctcctcaacgtcagggaatgagggctgggcattgccatccaggggttctgcgagagcattctgcgggtctttcctttctgtttcagaatcacacctgttctcacaagggataaatttgtcaccttcagtttttatttcaggaacttccaataggtcttttttatgatctgttaaaacatactttgggactctaggtggtttggtttcttctgagaagttggagccactgtcccagccattttctgcactttcagagttactttcattgtcatcagaggagcagaagggtggctgagaatcatcaatcttgtctcttccatcatcagaatgaatcagaaagcactcgtctgcttcatcgctctctgcttttaaagactggatgccactgtcatttaaattttcacttacagtctgaacagatacatttttttcaaatttccccaagtgcattaaagacttgaccatgagctcttgataacaagagtatctgtcttccttcctactggagttttcttgtgcagttgaaagaagactttcatccataggttttatcatgatttcctctgcggtagagtgaccatgtgtttccaaggggccatcgtcctctgtcctgtcactgcggtcttcttggcagtctgcttttgggctgtagtgtcggggcttcattagcagggatttccttttgttgactggaacccccaaagcctgatcttcagctgttctcttctttgccatggagcaatcataggcaacactgagctcctggattagtgaatccattggcacctcggttcctttagagcgagtacgcagcgttttatcttcagcctctgcatccatctataaacagatgtataaagtgatttcctagtacttgtacttgacgtcttttcttactggagcttacatcaggggcaataagcaggtctcttccacatcgccccagtgcacagatctggtaccttcttttaggctgaagaggaagtcctggaattgctctctttttctccaggtaacttgtatgtcaactcagtttgccctgctgtgtcagggggactaaataaatgactttgtcttatttagtgataaatcctgaaattcattctttcttgcagaaaatttctaccgtcctgccttctctaccctttgcagtatatcaaagtgctcagctttttaatcatagatttctgtgtttcttgtaggatttgaccagacattaaatagatgcttcttcaacttaagtcagcaactgtagttccttccctaaaagctactggatctgaactggagagtttccatcactcctttacctggcgaacgtctacaggtgtgtcgaaagttatcttttcctggatgtgttccaaaatgctcttatgctatttctcttaggatttctccacgctgccccattcagaaattttattattttctctagtattcccctgaggtcacattcagttaaaaacatcctgcccttctccctacaaaaaggttccatagaatc

SEQ ID NO: 18682 - RNA, 5157 nt, Homo sapiens
  source 1..5157: mol_type = other RNA
tgagtgtgtgtgtgtgagtgtgtgtgtatattttgtagcatttgaagttttgtggcaagatttctatcaaattgaatgttgtcttgtttcctatggtgggtgagacccaaggtgccagtgtttgaagtaatcattcagattggagtagcattttttcatgtgttactatattttccattcctttccagtcaacccagtaagataaatgctatttcaggggatatggtatctacaaaatttttcatttggatgtgtttgtatttgctaagtacaaatctacaccaatattgtcacttgtatattgtaccaacatatggcaggaaagcctggctggtcacaccaagtcttatttttcatcttgggatacgagttgccaacgatctgatatgacttgaaaaacaaacagacaaatctgcatcactaaaaaggcttatgtttctttaaaacatttcaaataaataattcatattaacgaaaaccgtccagccaagtcgaatactttgctgattgctatatttaattattgctaacaaattctgagcaggctgttttccagcatcctgtgcttttgtgagtgcggattccccactagtgggcgccatttgtcttcttattccttccgtgcagctcaccttaccgcaaattcatttataaatacaaaaatcagtgaaaggtgggggaagaagtgtgcaataaaaatcaaactcaactatagtgcagtccttagacaaggatttccttcaccctttcctgtttcctcattaaaacccagcaagaaagatgacttgagaatagcatttctatttaaatcctattggaaaataaattaataaacacacttgtaaaaatacggcagacttcaaaatgcagttaaaagataaaaaactctttgattagtaataaataaattataaaaatgtcacatttattttacatatactttacaaaaaaaaaaagagtacaatgaagaaataaaagaaaaacatatgaaaataaataagatctaataattgactgcattgcttttaatccaagaagtctatcatagtttttctttcctttttatatcagctggggaaaataaaattagtgcaatgttgcaaattgtaaatgcagtacggcaacctccacgccttagcagtacatgaacctctaacagatccatctggagtttactgctgttggtaacttctgttgcccggcagcgctgtgatcctacacatggatacccttcactgcctgtttgatactttccagtagagctttgcattccggggaatagtcccgttccagattgctgtacatatctgtgagtgtatttacatatgcttcaaaattctgctcactgataggtcccatctgtggaagctggatgtcagcaaggcttgaaatgagagcttggcttagacctgccagctctttcagcagactttcattgttctgttctatgagtttgttctcctcctctatcgtctttaagttgctctccatagatgtgatctgggtctgaagtttcatcatatctgcttcaattttaaggttggattcattcagttcctttatttcttcatccaaatgcctaatttcttcatcactctctattcccccagttgctttgagcttgatggtcatgagttcttcagaaaccttgccctttttgataacttgtgcattgagaggacatccagataagcttcggtgggtgacaaaaacattatttacatggcccagcccattgcagcctggcaagggacaatgtggtagctcttgtttgttcagtttccaggagagggaggctccattgagaggattctccttctgtctcttggcagccagaggacagccagaagctgtgcggtgtgatgtgtatttacctgatatgtgaccttggccatcacaccctatcacaggacatttcagttcagggtcttctttttcttccttggtaggggtcattttgacaccacctttccttgcacgagggcatccggacaagcttctgtgggaagcatagtttccagtcacgtgccccgagccatcgcagcctggggttggacacttaagctcctgagagttggcagccatgagggattttagagtcttatctgctaaaggacatccagaaacactgcgatgagatgcatagtttcctgtcacgtggccacttccatcacatcctggtgttggacaggtgattagttcctttttgagatctcttgcatgaagcttgggtttagggcttggtatagaggcctctccaggaaactttttttcctctaaattttctagagagctcactgggtctttctctttctcctcctctgtcttcccgtgagttttgctatagttgataggagtgtcccagccctcttggtcacaaagagcctgatagaatgctgcattgaccagaatgctgcttgttttgaatggggaagaggaaggagttggaatagaagtgttagaggaagttaggggtgcagacttgtccaggattcgattttttttcatgcttaagtccaatgtgccattttcatccacttctatttcggctcccttggcatgcagactctgtggcttgttggagaggatgtctgtggcttccctgcagcgggtggaaaggttcaggatggcagcagctgctgctatgtgggtgtcttcactacattgaccgtagctataagagctggcacggccagggctctgggtgtgggcgcctgcactaggcagtcgattaggaaatttcactggatttggaaaatgctttgattcaggaaatggtggtgtttttcgtccttgcactgtttgtatgagagggcgtttaccgaaaacttgggcatcaaaactggcataatcaaatggtacttttccaaacttctcttgttcttttgacactgtggctctgggagaggtgatggcttgtgacgggaaattgaattcaatttgcttcaccaaacttgtcctgtgggcctggtcaggacactgcccagtttggggagaatcaagctgatttttatcctgggacattgccaatttttcagctgcagcaattggacaaccagaaagactcctgtgggtgttgcggttgctgttcacatgaccccttcctgtgcatcccggcgtgggacacttgagcacattttcatgcatggcaagaatttccaggggaacccgcactttgtgggggcaccccgaaaggctgcggtggtgcgggtagagccctgtcacgtgtcccgtgccatcacatccagggatcgggcacttggtctccctcttttcaggccttggtgaatgtttattgttaaagatttgtcttccacccatgtcgataactttggtttgcctcctttcccctgctaggtgctccagcaggaacctatccagctctttgtaggtgttatggaaaacacaacctcgctcagcctgcagagcaattgcctgctccagcaaacttaaattccccttggccttttccaggtcactaccctcttccgtcattactgccaggctctcgctatcttcctcctcaacgtcagggaatgagggctgggcattgccatccaggggttctgcgagagcattctgcgggtctttcctttctgtttcagaatcacacctgttctcacaagggataaatttgtcaccttcagtttttatttcaggaacttccaataggtcttttttatgatctgttaaaacatactttgggactctaggtggtttggtttcttctgagaagttggagccactgtcccagccattttctgcactttcagagttactttcattgtcatcagaggagcagaagggtggctgagaatcatcaatcttgtctcttccatcatcagaatgaatcagaaagcactcgtctgcttcatcgctctctgcttttaaagactggatgccactgtcatttaaattttcacttacagtctgaacagatacatttttttcaaatttccccaagtgcattaaagacttgaccatgagctcttgataacaagagtatctgtcttccttcctactggagttttcttgtgcagttgaaagaagactttcatccataggttttatcatgatttcctctgcggtagagtgaccatgtgtttccaaggggccatcgtcctctgtcctgtcactgcggtcttcttggcagtctgcttttgggctgtagtgtcggggcttcattagcagggatttccttttgttgactggaacccccaaagcctgatcttcagctgttctcttctttgccatggagcaatcataggcaacactgagctcctggattagtgaatccattggcacctcggttcctttagagcgagtacgcagcgttttatcttcagcctctgcatccatctataaacagatgtataaagtgatttcctagtacttgtacttgacgtcttttcttactggagcttacatcaggggcaataagcaggtctcttccacatcgccccagtgcacagatctggtaccttcttttaggctgaagaggaagtcctggaattgctctctttttctccaggtaacttgtatgtcaactcagtttgccctgctgtgtcagggggactaaataaatgactttgtcttatttagtgataaatcctgaaattcattctttcttgcagaaaatttctaccgtcctgccttctctaccctttgcagtatatcaaagtgctcagctttttaatcatagatttctgtgtttcttgtaggatttgaccagacattaaatagatgcttcttcaacttaagtcagcaactgtagttccttccctaaaagctactggatctgaactggagagtttccatcactcctttacctggcgaacgtctacaggtgtgtcgaaagttatcttttcctggatgtgttccaaaatgctcttatgctatttctcttaggatttctccacgctgccccattcagaaattttattattttcttccacaactctgccaggcactggtttttgcgtgggatgatgccagcttctctcttcatgtggccttattaaaagccatggtttccgagatgtaaaacacccacagttacctcaattatttttctctccttacctctagtattcccctgaggtcacattcagttaaaaacatcctgcccttctccctacaaaaaggttccatagaatc

SEQ ID NO: 18683 - RNA, 4922 nt, Homo sapiens
  source 1..4922: mol_type = other RNA
tgagtgtgtgtgtgtgagtgtgtgtgtatattttgtagcatttgaagttttgtggcaagatttctatcaaattgaatgttgtcttgtttcctatggtgggtgagacccaaggtgccagtgtttgaagtaatcattcagattggagtagcattttttcatgtgttactatattttccattcctttccagtcaacccagtaagataaatgctatttcaggggatatggtatctacaaaatttttcatttggatgtgtttgtatttgctaagtacaaatctacaccaatattgtcacttgtatattgtaccaacatatggcaggaaagcctggctggtcacaccaagtcttatttttcatcttgggatacgagttgccaacgatctgatatgacttgaaaaacaaacagacaaatctgcatcactaaaaaggcttatgtttctttaaaacatttcaaataaataattcatattaacgaaaaccgtccagccaagtcgaatactttgctgattgctatatttaattattgctaacaaattctgagcaggctgttttccagcatcctgtgcttttgtgagtgcggattccccactagtgggcgccatttgtcttcttattccttccgtgcagctcaccttaccgcaaattcatttataaatacaaaaatcagtgaaaggtgggggaagaagtgtgcaataaaaatcaaactcaactatagtgcagtccttagacaaggatttccttcaccctttcctgtttcctcattaaaacccagcaagaaagatgacttgagaatagcatttctatttaaatcctattggaaaataaattaataaacacacttgtaaaaatacggcagacttcaaaatgcagttaaaagataaaaaactctttgattagtaataaataaattataaaaatgtcacatttattttacatatactttacaaaaaaaaaaagagtacaatgaagaaataaaagaaaaacatatgaaaataaataagatctaataattgactgcattgcttttaatccaagaagtctatcatagtttttctttcctttttatatcagctggggaaaataaaattagtgcaatgttgcaaattgtaaatgcagtacggcaacctccacgccttagcagtacatgaacctctaacagatccatctggagtttactgctgttggtaacttctgttgcccggcagcgctgtgatcctacacatggatacccttcactgcctgtttgatactttccagtagagctttgcattccggggaatagtcccgttccagattgctgtacatatctgtgagtgtatttacatatgcttcaaaattctgctcactgataggtcccatctgtggaagctggatgtcagcaaggcttgaaatgagagcttggcttagacctgccagctctttcagcagactttcattgttctgttctatgagtttgttctcctcctctatcgtctttaagttgctctccatagatgtgatctgggtctgaagtttcatcatatctgcttcaattttaaggttggattcattcagttcctttatttcttcatccaaatgcctaatttcttcatcactctctattcccccagttgctttgagcttgatggtcatgagttcttcagaaaccttgccctttttgataacttgtgcattgagaggacatccagataagcttcggtgggtgacaaaaacattatttacatggcccagcccattgcagcctggcaagggacaatgtggtagctcttgtttgttcagtttccaggagagggaggctccattgagaggattctccttctgtctcttggcagccagaggacagccagaagctgtgcggtgtgatgtgtatttacctgatatgtgaccttggccatcacaccctatcacaggacatttcagttcagggtcttctttttcttccttggtaggggtcattttgacaccacctttccttgcacgagggcatccggacaagcttctgtgggaagcatagtttccagtcacgtgccccgagccatcgcagcctggggttggacacttaagctcctgagagttggcagccatgagggattttagagtcttatctgctaaaggacatccagaaacactgcgatgagatgcatagtttcctgtcacgtggccacttccatcacatcctggtgttggacaggtgattagttcctttttgagatctcttgcatgaagcttgggtttagggcttggtatagaggcctctccaggaaactttttttcctctaaattttctagagagctcactgggtctttctctttctcctcctctgtcttcccgtgagttttgctatagttgataggagtgtcccagccctcttggtcacaaagagcctgatagaatgctgcattgaccagaatgctgcttgttttgaatggggaagaggaaggagttggaatagaagtgttagaggaagttaggggtgcagacttgtccaggattcgattttttttcatgcttaagtccaatgtgccattttcatccacttctatttcggctcccttggcatgcagactctgtggcttgttggagaggatgtctgtggcttccctgcagcgggtggaaaggttcaggatggcagcagctgctgctatgtgggtgtcttcactacattgaccgtagctataagagctggcacggccagggctctgggtgtgggcgcctgcactaggcagtcgattaggaaatttcactggatttggaaaatgctttgattcaggaaatggtggtgtttttcgtccttgcactgtttgtatgagagggcgtttaccgaaaacttgggcatcaaaactggcataatcaaatggtacttttccaaacttctcttgttcttttgacactgtggctctgggagaggtgatggcttgtgacgggaaattgaattcaatttgcttcaccaaacttgtcctgtgggcctggtcaggacactgcccagtttggggagaatcaagctgatttttatcctgggacattgccaatttttcagctgcagcaattggacaaccagaaagactcctgtgggtgttgcggttgctgttcacatgaccccttcctgtgcatcccggcgtgggacacttgagcacattttcatgcatggcaagaatttccaggggaacccgcactttgtgggggcaccccgaaaggctgcggtggtgcgggtagagccctgtcacgtgtcccgtgccatcacatccagggatcgggcacttggtctccctcttttcaggccttggtgaatgtttattgttaaagatttgtcttccacccatgtcgataactttggtttgcctcctttcccctgctaggtgctccagcaggaacctatccagctctttgtaggtgttatggaaaacacaacctcgctcagcctgcagagcaattgcctgctccagcaaacttaaattccccttggccttttccaggtcactaccctcttccgtcattactgccaggctctcgctatcttcctcctcaacgtcagggaatgagggctgggcattgccatccaggggttctgcgagagcattctgcgggtctttcctttctgtttcagaatcacacctgttctcacaagggataaatttgtcaccttcagtttttatttcaggaacttccaataggtcttttttatgatctgttaaaacatactttgggactctaggtggtttggtttcttctgagaagttggagccactgtcccagccattttctgcactttcagagttactttcattgtcatcagaggagcagaagggtggctgagaatcatcaatcttgtctcttccatcatcagaatgaatcagaaagcactcgtctgcttcatcgctctctgcttttaaagactggatgccactgtcatttaaattttcacttacagtctgaacagatacatttttttcaaatttccccaagtgcattaaagacttgaccatgagctcttgataacaagagtatctgtcttccttcctactggagttttcttgtgcagttgaaagaagactttcatccataggttttatcatgatttcctctgcggtagagtgaccatgtgtttccaaggggccatcgtcctctgtcctgtcactgcggtcttcttggcagtctgcttttgggctgtagtgtcggggcttcattagcagggatttccttttgttgactggaacccccaaagcctgatcttcagctgttctcttctttgccatggagcaatcataggcaacactgagctcctggattagtgaatccattggcacctcggttcctttagagcgagtacgcagcgttttatcttcagcctctgcatccatctataaacagatgtataaagtgatttcctagtacttgtacttgacgtcttttcttactggagcttacatcaggggcaataagcaggtctcttccacatcgccccagtgcacagatctggtaccttcttttaggctgaagaggaagtcctggaattgctctctttttctccaggtaacttgtatgtcaactcagtttgccctgctgtgtcagggggactaaataaatgactttgtcttatttagtgataaatcctgaaattcattctttcttgcagaaaatttctaccgtcctgccttctctaccctttgcagtatatcaaagtgctcagctttttaatcatagatttctgtgtttcttgtaggatttgaccagacattaaatagatgcttcttcaacttaagtcagcaactgtagttccttccctaaaagctactggatctgaactggagagtttccatcactcttttttgtttgtttccaaaacttatatttctctcctccctggtgggctgaacggaaacactaaagctgtttctttgaaaggtagttcccatgatatgac

SEQ ID NO: 18684 - RNA, 5056 nt, Homo sapiens
  source 1..5056: mol_type = other RNA
tgagtgtgtgtgtgtgagtgtgtgtgtatattttgtagcatttgaagttttgtggcaagatttctatcaaattgaatgttgtcttgtttcctatggtgggtgagacccaaggtgccagtgtttgaagtaatcattcagattggagtagcattttttcatgtgttactatattttccattcctttccagtcaacccagtaagataaatgctatttcaggggatatggtatctacaaaatttttcatttggatgtgtttgtatttgctaagtacaaatctacaccaatattgtcacttgtatattgtaccaacatatggcaggaaagcctggctggtcacaccaagtcttatttttcatcttgggatacgagttgccaacgatctgatatgacttgaaaaacaaacagacaaatctgcatcactaaaaaggcttatgtttctttaaaacatttcaaataaataattcatattaacgaaaaccgtccagccaagtcgaatactttgctgattgctatatttaattattgctaacaaattctgagcaggctgttttccagcatcctgtgcttttgtgagtgcggattccccactagtgggcgccatttgtcttcttattccttccgtgcagctcaccttaccgcaaattcatttataaatacaaaaatcagtgaaaggtgggggaagaagtgtgcaataaaaatcaaactcaactatagtgcagtccttagacaaggatttccttcaccctttcctgtttcctcattaaaacccagcaagaaagatgacttgagaatagcatttctatttaaatcctattggaaaataaattaataaacacacttgtaaaaatacggcagacttcaaaatgcagttaaaagataaaaaactctttgattagtaataaataaattataaaaatgtcacatttattttacatatactttacaaaaaaaaaaagagtacaatgaagaaataaaagaaaaacatatgaaaataaataagatctaataattgactgcattgcttttaatccaagaagtctatcatagtttttctttcctttttatatcagctggggaaaataaaattagtgcaatgttgcaaattgtaaatgcagtacggcaacctccacgccttagcagtacatgaacctctaacagatccatctggagtttactgctgttggtaacttctgttgcccggcagcgctgtgatcctacacatggatacccttcactgcctgtttgatactttccagtagagctttgcattccggggaatagtcccgttccagattgctgtacatatctgtgagtgtatttacatatgcttcaaaattctgctcactgataggtcccatctgtggaagctggatgtcagcaaggcttgaaatgagagcttggcttagacctgccagctctttcagcagactttcattgttctgttctatgagtttgttctcctcctctatcgtctttaagttgctctccatagatgtgatctgggtctgaagtttcatcatatctgcttcaattttaaggttggattcattcagttcctttatttcttcatccaaatgcctaatttcttcatcactctctattcccccagttgctttgagcttgatggtcatgagttcttcagaaaccttgccctttttgataacttgtgcattgagaggacatccagataagcttcggtgggtgacaaaaacattatttacatggcccagcccattgcagcctggcaagggacaatgtggtagctcttgtttgttcagtttccaggagagggaggctccattgagaggattctccttctgtctcttggcagccagaggacagccagaagctgtgcggtgtgatgtgtatttacctgatatgtgaccttggccatcacaccctatcacaggacatttcagttcagggtcttctttttcttccttggtaggggtcattttgacaccacctttccttgcacgagggcatccggacaagcttctgtgggaagcatagtttccagtcacgtgccccgagccatcgcagcctggggttggacacttaagctcctgagagttggcagccatgagggattttagagtcttatctgctaaaggacatccagaaacactgcgatgagatgcatagtttcctgtcacgtggccacttccatcacatcctggtgttggacaggtgattagttcctttttgagatctcttgcatgaagcttgggtttagggcttggtatagaggcctctccaggaaactttttttcctctaaattttctagagagctcactgggtctttctctttctcctcctctgtcttcccgtgagttttgctatagttgataggagtgtcccagccctcttggtcacaaagagcctgatagaatgctgcattgaccagaatgctgcttgttttgaatggggaagaggaaggagttggaatagaagtgttagaggaagttaggggtgcagacttgtccaggattcgattttttttcatgcttaagtccaatgtgccattttcatccacttctatttcggctcccttggcatgcagactctgtggcttgttggagaggatgtctgtggcttccctgcagcgggtggaaaggttcaggatggcagcagctgctgctatgtgggtgtcttcactacattgaccgtagctataagagctggcacggccagggctctgggtgtgggcgcctgcactaggcagtcgattaggaaatttcactggatttggaaaatgctttgattcaggaaatggtggtgtttttcgtccttgcactgtttgtatgagagggcgtttaccgaaaacttgggcatcaaaactggcataatcaaatggtacttttccaaacttctcttgttcttttgacactgtggctctgggagaggtgatggcttgtgacgggaaattgaattcaatttgcttcaccaaacttgtcctgtgggcctggtcaggacactgcccagtttggggagaatcaagctgatttttatcctgggacattgccaatttttcagctgcagcaattggacaaccagaaagactcctgtgggtgttgcggttgctgttcacatgaccccttcctgtgcatcccggcgtgggacacttgagcacattttcatgcatggcaagaatttccaggggaacccgcactttgtgggggcaccccgaaaggctgcggtggtgcgggtagagccctgtcacgtgtcccgtgccatcacatccagggatcgggcacttggtctccctcttttcaggccttggtgaatgtttattgttaaagatttgtcttccacccatgtcgataactttggtttgcctcctttcccctgctaggtgctccagcaggaacctatccagctctttgtaggtgttatggaaaacacaacctcgctcagcctgcagagcaattgcctgctccagcaaacttaaattccccttggccttttccaggtcactaccctcttccgtcattactgccaggctctcgctatcttcctcctcaacgtcagggaatgagggctgggcattgccatccaggggttctgcgagagcattctgcgggtctttcctttctgtttcagaatcacacctgttctcacaagggataaatttgtcaccttcagtttttatttcaggaacttccaataggtcttttttatgatctgttaaaacatactttgggactctaggtggtttggtttcttctgagaagttggagccactgtcccagccattttctgcactttcagagttactttcattgtcatcagaggagcagaagggtggctgagaatcatcaatcttgtctcttccatcatcagaatgaatcagaaagcactcgtctgcttcatcgctctctgcttttaaagactggatgccactgtcatttaaattttcacttacagtctgaacagatacatttttttcaaatttccccaagtgcattaaagacttgaccatgagctcttgataacaagagtatctgtcttccttcctactggagttttcttgtgcagttgaaagaagactttcatccataggttttatcatgatttcctctgcggtagagtgaccatgtgtttccaaggggccatcgtcctctgtcctgtcactgcggtcttcttggcagtctgcttttgggctgtagtgtcggggcttcattagcagggatttccttttgttgactggaacccccaaagcctgatcttcagctgttctcttctttgccatggagcaatcataggcaacactgagctcctggattagtgaatccattggcacctcggttcctttagagcgagtacgcagcgttttatcttcagcctctgcatccatctataacatgaacacaaagtcctgaggtcattcctataaacagatgtataaagtgatttcctagtacttgtacttgacgtcttttcttactggagcttacatcaggggcaataagcaggtctcttccacatcgccccagtgcacagatctggtaccttcttttaggctgaagaggaagtcctggaattgctctctttttctccaggtaacttgtatgtcaactcagtttgccctgctgtgtcagggggactaaataaatgactttgtcttatttagtgataaatcctgaaattcattctttcttgcagaaaatttctaccgtcctgccttctctaccctttgcagtatatcaaagtgctcagctttttaatcatagatttctgtgtttcttgtaggatttgaccagacattaaatagatgcttcttcaacttaagtcagcaactgtagttccttccctaaaagctactggatctgaactggagagtttccatcactcctttacctggcgaacgtctacaggtgtgtcgaaagttatcttttcctggatgtgttccaaaatgctcttatgctatttctcttaggatttctccacgctgccccattcagaaattttattattttctctagtattcccctgaggtcacattcagttaaaaacatcctgcccttctccctacaaaaaggttccatagaatc

SEQ ID NO: 18685 - RNA, 4886 nt, Homo sapiens
  source 1..4886: mol_type = other RNA
tgagtgtgtgtgtgtgagtgtgtgtgtatattttgtagcatttgaagttttgtggcaagatttctatcaaattgaatgttgtcttgtttcctatggtgggtgagacccaaggtgccagtgtttgaagtaatcattcagattggagtagcattttttcatgtgttactatattttccattcctttccagtcaacccagtaagataaatgctatttcaggggatatggtatctacaaaatttttcatttggatgtgtttgtatttgctaagtacaaatctacaccaatattgtcacttgtatattgtaccaacatatggcaggaaagcctggctggtcacaccaagtcttatttttcatcttgggatacgagttgccaacgatctgatatgacttgaaaaacaaacagacaaatctgcatcactaaaaaggcttatgtttctttaaaacatttcaaataaataattcatattaacgaaaaccgtccagccaagtcgaatactttgctgattgctatatttaattattgctaacaaattctgagcaggctgttttccagcatcctgtgcttttgtgagtgcggattccccactagtgggcgccatttgtcttcttattccttccgtgcagctcaccttaccgcaaattcatttataaatacaaaaatcagtgaaaggtgggggaagaagtgtgcaataaaaatcaaactcaactatagtgcagtccttagacaaggatttccttcaccctttcctgtttcctcattaaaacccagcaagaaagatgacttgagaatagcatttctatttaaatcctattggaaaataaattaataaacacacttgtaaaaatacggcagacttcaaaatgcagttaaaagataaaaaactctttgattagtaataaataaattataaaaatgtcacatttattttacatatactttacaaaaaaaaaaagagtacaatgaagaaataaaagaaaaacatatgaaaataaataagatctaataattgactgcattgcttttaatccaagaagtctatcatagtttttctttcctttttatatcagctggggaaaataaaattagtgcaatgttgcaaattgtaaatgcagtacggcaacctccacgccttagcagtacatgaacctctaacagatccatctggagtttactgctgttggtaacttctgttgcccggcagcgctgtgatcctacacatggatacccttcactgcctgtttgatactttccagtagagctttgcattccggggaatagtcccgttccagattgctgtacatatctgtgagtgtatttacatatgcttcaaaattctgctcactgataggtcccatctgtggaagctggatgtcagcaaggcttgaaatgagagcttggcttagacctgccagctctttcagcagactttcattgttctgttctatgagtttgttctcctcctctatcgtctttaagttgctctccatagatgtgatctgggtctgaagtttcatcatatctgcttcaattttaaggttggattcattcagttcctttatttcttcatccaaatgcctaatttcttcatcactctctattcccccagttgctttgagcttgatggtcatgagttcttcagaaaccttgccctttttgataacttgtgcattgagaggacatccagataagcttcggtgggtgacaaaaacattatttacatggcccagcccattgcagcctggcaagggacaatgtggtagctcttgtttgttcagtttccaggagagggaggctccattgagaggattctccttctgtctcttggcagccagaggacagccagaagctgtgcggtgtgatgtgtatttacctgatatgtgaccttggccatcacaccctatcacaggacatttcagttcagggtcttctttttcttccttggtaggggtcattttgacaccacctttccttgcacgagggcatccggacaagcttctgtgggaagcatagtttccagtcacgtgccccgagccatcgcagcctggggttggacacttaagctcctgagagttggcagccatgagggattttagagtcttatctgctaaaggacatccagaaacactgcgatgagatgcatagtttcctgtcacgtggccacttccatcacatcctggtgttggacaggtgattagttcctttttgagatctcttgcatgaagcttgggtttagggcttggtatagaggcctctccaggaaactttttttcctctaaattttctagagagctcactgggtctttctctttctcctcctctgtcttcccgtgagttttgctatagttgataggagtgtcccagccctcttggtcacaaagagcctgatagaatgctgcattgaccagaatgctgcttgttttgaatggggaagaggaaggagttggaatagaagtgttagaggaagttaggggtgcagacttgtccaggattcgattttttttcatgcttaagtccaatgtgccattttcatccacttctatttcggctcccttggcatgcagactctgtggcttgttggagaggatgtctgtggcttccctgcagcgggtggaaaggttcaggatggcagcagctgctgctatgtgggtgtcttcactacattgaccgtagctataagagctggcacggccagggctctgggtgtgggcgcctgcactaggcagtcgattaggaaatttcactggatttggaaaatgctttgattcaggaaatggtggtgtttttcgtccttgcactgtttgtatgagagggcgtttaccgaaaacttgggcatcaaaactggcataatcaaatggtacttttccaaacttctcttgttcttttgacactgtggctctgggagaggtgatggcttgtgacgggaaattgaattcaatttgcttcaccaaacttgtcctgtgggcctggtcaggacactgcccagtttggggagaatcaagctgatttttatcctgggacattgccaatttttcagctgcagcaattggacaaccagaaagactcctgtgggtgttgcggttgctgttcacatgaccccttcctgtgcatcccggcgtgggacacttgagcacattttcatgcatggcaagaatttccaggggaacccgcactttgtgggggcaccccgaaaggctgcggtggtgcgggtagagccctgtcacgtgtcccgtgccatcacatccagggatcgggcacttggtctccctcttttcaggccttggtgaatgtttattgttaaagatttgtcttccacccatgtcgataactttggtttgcctcctttcccctgctaggtgctccagcaggaacctatccagctctttgtaggtgttatggaaaacacaacctcgctcagcctgcagagcaattgcctgctccagcaaacttaaattccccttggccttttccaggtcactaccctcttccgtcattactgccaggctctcgctatcttcctcctcaacgtcagggaatgagggctgggcattgccatccaggggttctgcgagagcattctgcgggtctttcctttctgtttcagaatcacacctgttctcacaagggataaatttgtcaccttcagtttttatttcaggaacttccaataggtcttttttatgatctgttaaaacatactttgggactctaggtggtttggtttcttctgagaagttggagccactgtcccagccattttctgcactttcagagttactttcattgtcatcagaggagcagaagggtggctgagaatcatcaatcttgtctcttccatcatcagaatgaatcagaaagcactcgtctgcttcatcgctctctgcttttaaagactggatgccactgtcatttaaattttcacttacagtctgaacagatacatttttttcaaatttccccaagtgcattaaagacttgaccatgagctcttgataacaagagtatctgtcttccttcctactggagttttcttgtgcagttgaaagaagactttcatccataggttttatcatgatttcctctgcggtagagtgaccatgtgtttccaaggggccatcgtcctctgtcctgtcactgcggtcttcttggcagtctgcttttgggctgtagtgtcggggcttcattagcagggatttccttttgttgactggaacccccaaagcctgatcttcagctgttctcttctttgccatggagcaatcataggcaacactgagctcctggattagtgaatccattggcacctcggttcctttagagcgagtacgcagcgttttatcttcagcctctgcatccatctctctttttctccaggtaacttgtatgtcaactcagtttgccctgctgtgtcagggggactaaataaatgactttgtcttatttagtgataaatcctgaaattcattctttcttgcagaaaatttctaccgtcctgccttctctaccctttgcagtatatcaaagtgctcagctttttaatcatagatttctgtgtttcttgtaggatttgaccagacattaaatagatgcttcttcaacttaagtcagcaactgtagttcactagtaggcataacagtatttgtatttgtccttccagtcccttccctaaaagctactggatctgaactggagagtttccatcactccttagtcttgatatgagcacgcagacacataaaatggaattgtcacaatgcttcagggacactcacaaaattgggggctttttttgtttgtttccaaaacttatatttctctcctccctggtgggctgaacggaaacactaaagctgtttctttgaaaggtagttcccatgatatgac

SEQ ID NO: 18686 - RNA, 5240 nt, Homo sapiens
  source 1..5240: mol_type = other RNA
tgagtgtgtgtgtgtgagtgtgtgtgtatattttgtagcatttgaagttttgtggcaagatttctatcaaattgaatgttgtcttgtttcctatggtgggtgagacccaaggtgccagtgtttgaagtaatcattcagattggagtagcattttttcatgtgttactatattttccattcctttccagtcaacccagtaagataaatgctatttcaggggatatggtatctacaaaatttttcatttggatgtgtttgtatttgctaagtacaaatctacaccaatattgtcacttgtatattgtaccaacatatggcaggaaagcctggctggtcacaccaagtcttatttttcatcttgggatacgagttgccaacgatctgatatgacttgaaaaacaaacagacaaatctgcatcactaaaaaggcttatgtttctttaaaacatttcaaataaataattcatattaacgaaaaccgtccagccaagtcgaatactttgctgattgctatatttaattattgctaacaaattctgagcaggctgttttccagcatcctgtgcttttgtgagtgcggattccccactagtgggcgccatttgtcttcttattccttccgtgcagctcaccttaccgcaaattcatttataaatacaaaaatcagtgaaaggtgggggaagaagtgtgcaataaaaatcaaactcaactatagtgcagtccttagacaaggatttccttcaccctttcctgtttcctcattaaaacccagcaagaaagatgacttgagaatagcatttctatttaaatcctattggaaaataaattaataaacacacttgtaaaaatacggcagacttcaaaatgcagttaaaagataaaaaactctttgattagtaataaataaattataaaaatgtcacatttattttacatatactttacaaaaaaaaaaagagtacaatgaagaaataaaagaaaaacatatgaaaataaataagatctaataattgactgcattgcttttaatccaagaagtctatcatagtttttctttcctttttatatcagctggggaaaataaaattagtgcaatgttgcaaattgtaaatgcagtacggcaacctccacgccttagcagtacatgaacctctaacagatccatctggagtttactgctgttggtaacttctgttgcccggcagcgctgtgatcctacacatggatacccttcactgcctgtttgatactttccagtagagctttgcattccggggaatagtcccgttccagattgctgtacatatctgtgagtgtatttacatatgcttcaaaattctgctcactgataggtcccatctgtggaagctggatgtcagcaaggcttgaaatgagagcttggcttagacctgccagctctttcagcagactttcattgttctgttctatgagtttgttctcctcctctatcgtctttaagttgctctccatagatgtgatctgggtctgaagtttcatcatatctgcttcaattttaaggttggattcattcagttcctttatttcttcatccaaatgcctaatttcttcatcactctctattcccccagttgctttgagcttgatggtcatgagttcttcagaaaccttgccctttttgataacttgtgcattgagaggacatccagataagcttcggtgggtgacaaaaacattatttacatggcccagcccattgcagcctggcaagggacaatgtggtagctcttgtttgttcagtttccaggagagggaggctccattgagaggattctccttctgtctcttggcagccagaggacagccagaagctgtgcggtgtgatgtgtatttacctgatatgtgaccttggccatcacaccctatcacaggacatttcagttcagggtcttctttttcttccttggtaggggtcattttgacaccacctttccttgcacgagggcatccggacaagcttctgtgggaagcatagtttccagtcacgtgccccgagccatcgcagcctggggttggacacttaagctcctgagagttggcagccatgagggattttagagtcttatctgctaaaggacatccagaaacactgcgatgagatgcatagtttcctgtcacgtggccacttccatcacatcctggtgttggacaggtgattagttcctttttgagatctcttgcatgaagcttgggtttagggcttggtatagaggcctctccaggaaactttttttcctctaaattttctagagagctcactgggtctttctctttctcctcctctgtcttcccgtgagttttgctatagttgataggagtgtcccagccctcttggtcacaaagagcctgatagaatgctgcattgaccagaatgctgcttgttttgaatggggaagaggaaggagttggaatagaagtgttagaggaagttaggggtgcagacttgtccaggattcgattttttttcatgcttaagtccaatgtgccattttcatccacttctatttcggctcccttggcatgcagactctgtggcttgttggagaggatgtctgtggcttccctgcagcgggtggaaaggttcaggatggcagcagctgctgctatgtgggtgtcttcactacattgaccgtagctataagagctggcacggccagggctctgggtgtgggcgcctgcactaggcagtcgattaggaaatttcactggatttggaaaatgctttgattcaggaaatggtggtgtttttcgtccttgcactgtttgtatgagagggcgtttaccgaaaacttgggcatcaaaactggcataatcaaatggtacttttccaaacttctcttgttcttttgacactgtggctctgggagaggtgatggcttgtgacgggaaattgaattcaatttgcttcaccaaacttgtcctgtgggcctggtcaggacactgcccagtttggggagaatcaagctgatttttatcctgggacattgccaatttttcagctgcagcaattggacaaccagaaagactcctgtgggtgttgcggttgctgttcacatgaccccttcctgtgcatcccggcgtgggacacttgagcacattttcatgcatggcaagaatttccaggggaacccgcactttgtgggggcaccccgaaaggctgcggtggtgcgggtagagccctgtcacgtgtcccgtgccatcacatccagggatcgggcacttggtctccctcttttcaggccttggtgaatgtttattgttaaagatttgtcttccacccatgtcgataactttggtttgcctcctttcccctgctaggtgctccagcaggaacctatccagctctttgtaggtgttatggaaaacacaacctcgctcagcctgcagagcaattgcctgctccagcaaacttaaattccccttggccttttccaggtcactaccctcttccgtcattactgccaggctctcgctatcttcctcctcaacgtcagggaatgagggctgggcattgccatccaggggttctgcgagagcattctgcgggtctttcctttctgtttcagaatcacacctgttctcacaagggataaatttgtcaccttcagtttttatttcaggaacttccaataggtcttttttatgatctgttaaaacatactttgggactctaggtggtttggtttcttctgagaagttggagccactgtcccagccattttctgcactttcagagttactttcattgtcatcagaggagcagaagggtggctgagaatcatcaatcttgtctcttccatcatcagaatgaatcagaaagcactcgtctgcttcatcgctctctgcttttaaagactggatgccactgtcatttaaattttcacttacagtctgaacagatacatttttttcaaatttccccaagtgcattaaagacttgaccatgagctcttgataacaagagtatctgtcttccttcctactggagttttcttgtgcagttgaaagaagactttcatccataggttttatcatgatttcctctgcggtagagtgaccatgtgtttccaaggggccatcgtcctctgtcctgtcactgcggtcttcttggcagtctgcttttgggctgtagtgtcggggcttcattagcagggatttccttttgttgactggaacccccaaagcctgatcttcagctgttctcttctttgccatggagcaatcataggcaacactgagctcctggattagtgaatccattggcacctcggttcctttagagcgagtacgcagcgttttatcttcagcctctgcatccatctctctttttctccaggtaacttgtatgtcaactcagtttgccctgctgtgtcagggggactaaataaatgactttgtcttatttagtgataaatcctgaaattcattctttcttgcagaaaatttctaccgtcctgccttctctaccctttgcagtatatcaaagtgctcagctttttaatcatagatttctgtgtttcttgtaggatttgaccagacattaaatagatgcttcttcaacttaagtcagcaactgtagttccttccctaaaagctactggatctgaactggagagtttccatcactccggtgcctcctagcctttgttctgcctctcacgctgacatcagggaagcagtgatgtagaataaagcaggggtgggctaggttagtccagtgtttgtgtcgttgtgtggtgtgcagggacactctgtgatactctagtgagctgctaagctttttttgtaggctttgtgtcatttacttaacgaccaatctcattagctgccagggtacaatgggctgatgcattttctatgtacatactccacacagtgaccctcaaggttgccgaaggtctatttaatcagacaaatgctgaatatatttgcagtaaatcactaaaaaaataaaaaaaattagaatactgaggtatcttacgggcttaatatttcctggtggttatttgcaggtaataaaatacatgcatatttagcccaaacaacgatagagcaggtggagatgaattgtctggtttgcactggtgaccttaattttaggaaactttcagatcaaagatattttctcttagcaaggagcccagatttgaaatttaatttctgtcttagtttaatcatattagcacaacaaaaaagaattg

SEQ ID NO: 18687 - RNA, 4912 nt, Homo sapiens
  source 1..4912: mol_type = other RNA
tgagtgtgtgtgtgtgagtgtgtgtgtatattttgtagcatttgaagttttgtggcaagatttctatcaaattgaatgttgtcttgtttcctatggtgggtgagacccaaggtgccagtgtttgaagtaatcattcagattggagtagcattttttcatgtgttactatattttccattcctttccagtcaacccagtaagataaatgctatttcaggggatatggtatctacaaaatttttcatttggatgtgtttgtatttgctaagtacaaatctacaccaatattgtcacttgtatattgtaccaacatatggcaggaaagcctggctggtcacaccaagtcttatttttcatcttgggatacgagttgccaacgatctgatatgacttgaaaaacaaacagacaaatctgcatcactaaaaaggcttatgtttctttaaaacatttcaaataaataattcatattaacgaaaaccgtccagccaagtcgaatactttgctgattgctatatttaattattgctaacaaattctgagcaggctgttttccagcatcctgtgcttttgtgagtgcggattccccactagtgggcgccatttgtcttcttattccttccgtgcagctcaccttaccgcaaattcatttataaatacaaaaatcagtgaaaggtgggggaagaagtgtgcaataaaaatcaaactcaactatagtgcagtccttagacaaggatttccttcaccctttcctgtttcctcattaaaacccagcaagaaagatgacttgagaatagcatttctatttaaatcctattggaaaataaattaataaacacacttgtaaaaatacggcagacttcaaaatgcagttaaaagataaaaaactctttgattagtaataaataaattataaaaatgtcacatttattttacatatactttacaaaaaaaaaaagagtacaatgaagaaataaaagaaaaacatatgaaaataaataagatctaataattgactgcattgcttttaatccaagaagtctatcatagtttttctttcctttttatatcagctggggaaaataaaattagtgcaatgttgcaaattgtaaatgcagtacggcaacctccacgccttagcagtacatgaacctctaacagatccatctggagtttactgctgttggtaacttctgttgcccggcagcgctgtgatcctacacatggatacccttcactgcctgtttgatactttccagtagagctttgcattccggggaatagtcccgttccagattgctgtacatatctgtgagtgtatttacatatgcttcaaaattctgctcactgataggtcccatctgtggaagctggatgtcagcaaggcttgaaatgagagcttggcttagacctgccagctctttcagcagactttcattgttctgttctatgagtttgttctcctcctctatcgtctttaagttgctctccatagatgtgatctgggtctgaagtttcatcatatctgcttcaattttaaggttggattcattcagttcctttatttcttcatccaaatgcctaatttcttcatcactctctattcccccagttgctttgagcttgatggtcatgagttcttcagaaaccttgccctttttgataacttgtgcattgagaggacatccagataagcttcggtgggtgacaaaaacattatttacatggcccagcccattgcagcctggcaagggacaatgtggtagctcttgtttgttcagtttccaggagagggaggctccattgagaggattctccttctgtctcttggcagccagaggacagccagaagctgtgcggtgtgatgtgtatttacctgatatgtgaccttggccatcacaccctatcacaggacatttcagttcagggtcttctttttcttccttggtaggggtcattttgacaccacctttccttgcacgagggcatccggacaagcttctgtgggaagcatagtttccagtcacgtgccccgagccatcgcagcctggggttggacacttaagctcctgagagttggcagccatgagggattttagagtcttatctgctaaaggacatccagaaacactgcgatgagatgcatagtttcctgtcacgtggccacttccatcacatcctggtgttggacaggtgattagttcctttttgagatctcttgcatgaagcttgggtttagggcttggtatagaggcctctccaggaaactttttttcctctaaattttctagagagctcactgggtctttctctttctcctcctctgtcttcccgtgagttttgctatagttgataggagtgtcccagccctcttggtcacaaagagcctgatagaatgctgcattgaccagaatgctgcttgttttgaatggggaagaggaaggagttggaatagaagtgttagaggaagttaggggtgcagacttgtccaggattcgattttttttcatgcttaagtccaatgtgccattttcatccacttctatttcggctcccttggcatgcagactctgtggcttgttggagaggatgtctgtggcttccctgcagcgggtggaaaggttcaggatggcagcagctgctgctatgtgggtgtcttcactacattgaccgtagctataagagctggcacggccagggctctgggtgtgggcgcctgcactaggcagtcgattaggaaatttcactggatttggaaaatgctttgattcaggaaatggtggtgtttttcgtccttgcactgtttgtatgagagggcgtttaccgaaaacttgggcatcaaaactggcataatcaaatggtacttttccaaacttctcttgttcttttgacactgtggctctgggagaggtgatggcttgtgacgggaaattgaattcaatttgcttcaccaaacttgtcctgtgggcctggtcaggacactgcccagtttggggagaatcaagctgatttttatcctgggacattgccaatttttcagctgcagcaattggacaaccagaaagactcctgtgggtgttgcggttgctgttcacatgaccccttcctgtgcatcccggcgtgggacacttgagcacattttcatgcatggcaagaatttccaggggaacccgcactttgtgggggcaccccgaaaggctgcggtggtgcgggtagagccctgtcacgtgtcccgtgccatcacatccagggatcgggcacttggtctccctcttttcaggccttggtgaatgtttattgttaaagatttgtcttccacccatgtcgataactttggtttgcctcctttcccctgctaggtgctccagcaggaacctatccagctctttgtaggtgttatggaaaacacaacctcgctcagcctgcagagcaattgcctgctccagcaaacttaaattccccttggccttttccaggtcactaccctcttccgtcattactgccaggctctcgctatcttcctcctcaacgtcagggaatgagggctgggcattgccatccaggggttctgcgagagcattctgcgggtctttcctttctgtttcagaatcacacctgttctcacaagggataaatttgtcaccttcagtttttatttcaggaacttccaataggtcttttttatgatctgttaaaacatactttgggactctaggtggtttggtttcttctgagaagttggagccactgtcccagccattttctgcactttcagagttactttcattgtcatcagaggagcagaagggtggctgagaatcatcaatcttgtctcttccatcatcagaatgaatcagaaagcactcgtctgcttcatcgctctctgcttttaaagactggatgccactgtcatttaaattttcacttacagtctgaacagatacatttttttcaaatttccccaagtgcattaaagacttgaccatgagctcttgataacaagagtatctgtcttccttcctactggagttttcttgtgcagttgaaagaagactttcatccataggttttatcatgatttcctctgcggtagagtgaccatgtgtttccaaggggccatcgtcctctgtcctgtcactgcggtcttcttggcagtctgcttttgggctgtagtgtcggggcttcattagcagggatttccttttgttgactggaacccccaaagcctgatcttcagctgttctcttctttgccatggagcaatcataggcaacactgagctcctggattagtgaatccattggcacctcggttcctttagagcgagtacgcagcgttttatcttcagcctctgcatccatctctctttttctccaggtaacttgtatgtcaactcagtttgccctgctgtgtcagggggactaaataaatgactttgtcttatttagtgataaatcctgaaattcattctttcttgcagaaaatttctaccgtcctgccttctctaccctttgcagtatatcaaagtgctcagctttttaatcatagatttctgtgtttcttgtaggatttgaccagacattaaatagatgcttcttcaacttaagtcagcaactgtagttccttccctaaaagctactggatctgaactggagagtttccatcactccttagtcttgatatgagcacgcagacacataaaatggaattgtcacaatgcttcagggacactcacaaaattgggggctctgaatgtcttgtaacaatatcatcctctcttgaactaaacatcctctgaatacacaaatctaaggcagacagacatttcagcaaggcaaataagactttctggcaacttcctgttgccatatttctctcaaaggatcctgcaatgttacacttcaatcctgcaaa

SEQ ID NO: 18688 - RNA, 4946 nt, Homo sapiens
  source 1..4946: mol_type = other RNA
tgagtgtgtgtgtgtgagtgtgtgtgtatattttgtagcatttgaagttttgtggcaagatttctatcaaattgaatgttgtcttgtttcctatggtgggtgagacccaaggtgccagtgtttgaagtaatcattcagattggagtagcattttttcatgtgttactatattttccattcctttccagtcaacccagtaagataaatgctatttcaggggatatggtatctacaaaatttttcatttggatgtgtttgtatttgctaagtacaaatctacaccaatattgtcacttgtatattgtaccaacatatggcaggaaagcctggctggtcacaccaagtcttatttttcatcttgggatacgagttgccaacgatctgatatgacttgaaaaacaaacagacaaatctgcatcactaaaaaggcttatgtttctttaaaacatttcaaataaataattcatattaacgaaaaccgtccagccaagtcgaatactttgctgattgctatatttaattattgctaacaaattctgagcaggctgttttccagcatcctgtgcttttgtgagtgcggattccccactagtgggcgccatttgtcttcttattccttccgtgcagctcaccttaccgcaaattcatttataaatacaaaaatcagtgaaaggtgggggaagaagtgtgcaataaaaatcaaactcaactatagtgcagtccttagacaaggatttccttcaccctttcctgtttcctcattaaaacccagcaagaaagatgacttgagaatagcatttctatttaaatcctattggaaaataaattaataaacacacttgtaaaaatacggcagacttcaaaatgcagttaaaagataaaaaactctttgattagtaataaataaattataaaaatgtcacatttattttacatatactttacaaaaaaaaaaagagtacaatgaagaaataaaagaaaaacatatgaaaataaataagatctaataattgactgcattgcttttaatccaagaagtctatcatagtttttctttcctttttatatcagctggggaaaataaaattagtgcaatgttgcaaattgtaaatgcagtacggcaacctccacgccttagcagtacatgaacctctaacagatccatctggagtttactgctgttggtaacttctgttgcccggcagcgctgtgatcctacacatggatacccttcactgcctgtttgatactttccagtagagctttgcattccggggaatagtcccgttccagattgctgtacatatctgtgagtgtatttacatatgcttcaaaattctgctcactgataggtcccatctgtggaagctggatgtcagcaaggcttgaaatgagagcttggcttagacctgccagctctttcagcagactttcattgttctgttctatgagtttgttctcctcctctatcgtctttaagttgctctccatagatgtgatctgggtctgaagtttcatcatatctgcttcaattttaaggttggattcattcagttcctttatttcttcatccaaatgcctaatttcttcatcactctctattcccccagttgctttgagcttgatggtcatgagttcttcagaaaccttgccctttttgataacttgtgcattgagaggacatccagataagcttcggtgggtgacaaaaacattatttacatggcccagcccattgcagcctggcaagggacaatgtggtagctcttgtttgttcagtttccaggagagggaggctccattgagaggattctccttctgtctcttggcagccagaggacagccagaagctgtgcggtgtgatgtgtatttacctgatatgtgaccttggccatcacaccctatcacaggacatttcagttcagggtcttctttttcttccttggtaggggtcattttgacaccacctttccttgcacgagggcatccggacaagcttctgtgggaagcatagtttccagtcacgtgccccgagccatcgcagcctggggttggacacttaagctcctgagagttggcagccatgagggattttagagtcttatctgctaaaggacatccagaaacactgcgatgagatgcatagtttcctgtcacgtggccacttccatcacatcctggtgttggacaggtgattagttcctttttgagatctcttgcatgaagcttgggtttagggcttggtatagaggcctctccaggaaactttttttcctctaaattttctagagagctcactgggtctttctctttctcctcctctgtcttcccgtgagttttgctatagttgataggagtgtcccagccctcttggtcacaaagagcctgatagaatgctgcattgaccagaatgctgcttgttttgaatggggaagaggaaggagttggaatagaagtgttagaggaagttaggggtgcagacttgtccaggattcgattttttttcatgcttaagtccaatgtgccattttcatccacttctatttcggctcccttggcatgcagactctgtggcttgttggagaggatgtctgtggcttccctgcagcgggtggaaaggttcaggatggcagcagctgctgctatgtgggtgtcttcactacattgaccgtagctataagagctggcacggccagggctctgggtgtgggcgcctgcactaggcagtcgattaggaaatttcactggatttggaaaatgctttgattcaggaaatggtggtgtttttcgtccttgcactgtttgtatgagagggcgtttaccgaaaacttgggcatcaaaactggcataatcaaatggtacttttccaaacttctcttgttcttttgacactgtggctctgggagaggtgatggcttgtgacgggaaattgaattcaatttgcttcaccaaacttgtcctgtgggcctggtcaggacactgcccagtttggggagaatcaagctgatttttatcctgggacattgccaatttttcagctgcagcaattggacaaccagaaagactcctgtgggtgttgcggttgctgttcacatgaccccttcctgtgcatcccggcgtgggacacttgagcacattttcatgcatggcaagaatttccaggggaacccgcactttgtgggggcaccccgaaaggctgcggtggtgcgggtagagccctgtcacgtgtcccgtgccatcacatccagggatcgggcacttggtctccctcttttcaggccttggtgaatgtttattgttaaagatttgtcttccacccatgtcgataactttggtttgcctcctttcccctgctaggtgctccagcaggaacctatccagctctttgtaggtgttatggaaaacacaacctcgctcagcctgcagagcaattgcctgctccagcaaacttaaattccccttggccttttccaggtcactaccctcttccgtcattactgccaggctctcgctatcttcctcctcaacgtcagggaatgagggctgggcattgccatccaggggttctgcgagagcattctgcgggtctttcctttctgtttcagaatcacacctgttctcacaagggataaatttgtcaccttcagtttttatttcaggaacttccaataggtcttttttatgatctgttaaaacatactttgggactctaggtggtttggtttcttctgagaagttggagccactgtcccagccattttctgcactttcagagttactttcattgtcatcagaggagcagaagggtggctgagaatcatcaatcttgtctcttccatcatcagaatgaatcagaaagcactcgtctgcttcatcgctctctgcttttaaagactggatgccactgtcatttaaattttcacttacagtctgaacagatacatttttttcaaatttccccaagtgcattaaagacttgaccatgagctcttgataacaagagtatctgtcttccttcctactggagttttcttgtgcagttgaaagaagactttcatccataggttttatcatgatttcctctgcggtagagtgaccatgtgtttccaaggggccatcgtcctctgtcctgtcactgcggtcttcttggcagtctgcttttgggctgtagtgtcggggcttcattagcagggatttccttttgttgactggaacccccaaagcctgatcttcagctgttctcttctttgccatggagcaatcataggcaacactgagctcctggattagtgaatccattggcacctcggttcctttagagcgagtacgcagcgttttatcttcagcctctgcatccatctctctttttctccaggtaacttgtatgtcaactcagtttgccctgctgtgtcagggggactaaataaatgactttgtcttatttagtgataaatcctgaaattcattctttcttgcagaaaatttctaccgtcctgccttctctaccctttgcagtatatcaaagtgctcagctttttaatcatagatttctgtgtttcttgtaggatttgaccagacattaaatagatgcttcttcaacttaagtcagcaactgtagttccttccctaaaagctactggatctgaactggagagtttccatcactccttagtcttgatatgagcacgcagacacataaaatggaattgtcacaatgcttcagggacactcacaaaattgggggctctttacctggcgaacgtctacaggtgtgtcgaaagttatcttttcctggatgtgttccaaaatgctcttatgctatttctcttaggatttctccacgctgccccattcagaaattttattattttctctagtattcccctgaggtcacattcagttaaaaacatcctgcccttctccctacaaaaaggttccatagaatc

SEQ ID NO: 18689 - RNA, 5080 nt, Homo sapiens
  source 1..5080: mol_type = other RNA
tgagtgtgtgtgtgtgagtgtgtgtgtatattttgtagcatttgaagttttgtggcaagatttctatcaaattgaatgttgtcttgtttcctatggtgggtgagacccaaggtgccagtgtttgaagtaatcattcagattggagtagcattttttcatgtgttactatattttccattcctttccagtcaacccagtaagataaatgctatttcaggggatatggtatctacaaaatttttcatttggatgtgtttgtatttgctaagtacaaatctacaccaatattgtcacttgtatattgtaccaacatatggcaggaaagcctggctggtcacaccaagtcttatttttcatcttgggatacgagttgccaacgatctgatatgacttgaaaaacaaacagacaaatctgcatcactaaaaaggcttatgtttctttaaaacatttcaaataaataattcatattaacgaaaaccgtccagccaagtcgaatactttgctgattgctatatttaattattgctaacaaattctgagcaggctgttttccagcatcctgtgcttttgtgagtgcggattccccactagtgggcgccatttgtcttcttattccttccgtgcagctcaccttaccgcaaattcatttataaatacaaaaatcagtgaaaggtgggggaagaagtgtgcaataaaaatcaaactcaactatagtgcagtccttagacaaggatttccttcaccctttcctgtttcctcattaaaacccagcaagaaagatgacttgagaatagcatttctatttaaatcctattggaaaataaattaataaacacacttgtaaaaatacggcagacttcaaaatgcagttaaaagataaaaaactctttgattagtaataaataaattataaaaatgtcacatttattttacatatactttacaaaaaaaaaaagagtacaatgaagaaataaaagaaaaacatatgaaaataaataagatctaataattgactgcattgcttttaatccaagaagtctatcatagtttttctttcctttttatatcagctggggaaaataaaattagtgcaatgttgcaaattgtaaatgcagtacggcaacctccacgccttagcagtacatgaacctctaacagatccatctggagtttactgctgttggtaacttctgttgcccggcagcgctgtgatcctacacatggatacccttcactgcctgtttgatactttccagtagagctttgcattccggggaatagtcccgttccagattgctgtacatatctgtgagtgtatttacatatgcttcaaaattctgctcactgataggtcccatctgtggaagctggatgtcagcaaggcttgaaatgagagcttggcttagacctgccagctctttcagcagactttcattgttctgttctatgagtttgttctcctcctctatcgtctttaagttgctctccatagatgtgatctgggtctgaagtttcatcatatctgcttcaattttaaggttggattcattcagttcctttatttcttcatccaaatgcctaatttcttcatcactctctattcccccagttgctttgagcttgatggtcatgagttcttcagaaaccttgccctttttgataacttgtgcattgagaggacatccagataagcttcggtgggtgacaaaaacattatttacatggcccagcccattgcagcctggcaagggacaatgtggtagctcttgtttgttcagtttccaggagagggaggctccattgagaggattctccttctgtctcttggcagccagaggacagccagaagctgtgcggtgtgatgtgtatttacctgatatgtgaccttggccatcacaccctatcacaggacatttcagttcagggtcttctttttcttccttggtaggggtcattttgacaccacctttccttgcacgagggcatccggacaagcttctgtgggaagcatagtttccagtcacgtgccccgagccatcgcagcctggggttggacacttaagctcctgagagttggcagccatgagggattttagagtcttatctgctaaaggacatccagaaacactgcgatgagatgcatagtttcctgtcacgtggccacttccatcacatcctggtgttggacaggtgattagttcctttttgagatctcttgcatgaagcttgggtttagggcttggtatagaggcctctccaggaaactttttttcctctaaattttctagagagctcactgggtctttctctttctcctcctctgtcttcccgtgagttttgctatagttgataggagtgtcccagccctcttggtcacaaagagcctgatagaatgctgcattgaccagaatgctgcttgttttgaatggggaagaggaaggagttggaatagaagtgttagaggaagttaggggtgcagacttgtccaggattcgattttttttcatgcttaagtccaatgtgccattttcatccacttctatttcggctcccttggcatgcagactctgtggcttgttggagaggatgtctgtggcttccctgcagcgggtggaaaggttcaggatggcagcagctgctgctatgtgggtgtcttcactacattgaccgtagctataagagctggcacggccagggctctgggtgtgggcgcctgcactaggcagtcgattaggaaatttcactggatttggaaaatgctttgattcaggaaatggtggtgtttttcgtccttgcactgtttgtatgagagggcgtttaccgaaaacttgggcatcaaaactggcataatcaaatggtacttttccaaacttctcttgttcttttgacactgtggctctgggagaggtgatggcttgtgacgggaaattgaattcaatttgcttcaccaaacttgtcctgtgggcctggtcaggacactgcccagtttggggagaatcaagctgatttttatcctgggacattgccaatttttcagctgcagcaattggacaaccagaaagactcctgtgggtgttgcggttgctgttcacatgaccccttcctgtgcatcccggcgtgggacacttgagcacattttcatgcatggcaagaatttccaggggaacccgcactttgtgggggcaccccgaaaggctgcggtggtgcgggtagagccctgtcacgtgtcccgtgccatcacatccagggatcgggcacttggtctccctcttttcaggccttggtgaatgtttattgttaaagatttgtcttccacccatgtcgataactttggtttgcctcctttcccctgctaggtgctccagcaggaacctatccagctctttgtaggtgttatggaaaacacaacctcgctcagcctgcagagcaattgcctgctccagcaaacttaaattccccttggccttttccaggtcactaccctcttccgtcattactgccaggctctcgctatcttcctcctcaacgtcagggaatgagggctgggcattgccatccaggggttctgcgagagcattctgcgggtctttcctttctgtttcagaatcacacctgttctcacaagggataaatttgtcaccttcagtttttatttcaggaacttccaataggtcttttttatgatctgttaaaacatactttgggactctaggtggtttggtttcttctgagaagttggagccactgtcccagccattttctgcactttcagagttactttcattgtcatcagaggagcagaagggtggctgagaatcatcaatcttgtctcttccatcatcagaatgaatcagaaagcactcgtctgcttcatcgctctctgcttttaaagactggatgccactgtcatttaaattttcacttacagtctgaacagatacatttttttcaaatttccccaagtgcattaaagacttgaccatgagctcttgataacaagagtatctgtcttccttcctactggagttttcttgtgcagttgaaagaagactttcatccataggttttatcatgatttcctctgcggtagagtgaccatgtgtttccaaggggccatcgtcctctgtcctgtcactgcggtcttcttggcagtctgcttttgggctgtagtgtcggggcttcattagcagggatttccttttgttgactggaacccccaaagcctgatcttcagctgttctcttctttgccatggagcaatcataggcaacactgagctcctggattagtgaatccattggcacctcggttcctttagagcgagtacgcagcgttttatcttcagcctctgcatccatctctctttttctccaggtaacttgtatgtcaactcagtttgccctgctgtgtcagggggactaaataaatgactttgtcttatttagtgataaatcctgaaattcattctttcttgcagaaaatttctaccgtcctgccttctctaccctttgcagtatatcaaagtgctcagctttttaatcatagatttctgtgtttcttgtaggatttgaccagacattaaatagatgcttcttcaacttaagtcagcaactgtagttccttccctaaaagctactggatctgaactggagagtttccatcactccttagtcttgatatgagcacgcagacacataaaatggaattgtcacaatgcttcagggacactcacaaaattgggggctctttacctggcgaacgtctacaggtgtgtcgaaagttatcttttcctggatgtgttccaaaatgctcttatgctatttctcttaggatttctccacgctgccccattcagaaattttattattttcttccacaactctgccaggcactggtttttgcgtgggatgatgccagcttctctcttcatgtggccttattaaaagccatggtttccgagatgtaaaacacccacagttacctcaattatttttctctccttacctctagtattcccctgaggtcacattcagttaaaaacatcctgcccttctccctacaaaaaggttccatagaatc

SEQ ID NO: 18690 - RNA, 4845 nt, Homo sapiens
  source 1..4845: mol_type = other RNA
tgagtgtgtgtgtgtgagtgtgtgtgtatattttgtagcatttgaagttttgtggcaagatttctatcaaattgaatgttgtcttgtttcctatggtgggtgagacccaaggtgccagtgtttgaagtaatcattcagattggagtagcattttttcatgtgttactatattttccattcctttccagtcaacccagtaagataaatgctatttcaggggatatggtatctacaaaatttttcatttggatgtgtttgtatttgctaagtacaaatctacaccaatattgtcacttgtatattgtaccaacatatggcaggaaagcctggctggtcacaccaagtcttatttttcatcttgggatacgagttgccaacgatctgatatgacttgaaaaacaaacagacaaatctgcatcactaaaaaggcttatgtttctttaaaacatttcaaataaataattcatattaacgaaaaccgtccagccaagtcgaatactttgctgattgctatatttaattattgctaacaaattctgagcaggctgttttccagcatcctgtgcttttgtgagtgcggattccccactagtgggcgccatttgtcttcttattccttccgtgcagctcaccttaccgcaaattcatttataaatacaaaaatcagtgaaaggtgggggaagaagtgtgcaataaaaatcaaactcaactatagtgcagtccttagacaaggatttccttcaccctttcctgtttcctcattaaaacccagcaagaaagatgacttgagaatagcatttctatttaaatcctattggaaaataaattaataaacacacttgtaaaaatacggcagacttcaaaatgcagttaaaagataaaaaactctttgattagtaataaataaattataaaaatgtcacatttattttacatatactttacaaaaaaaaaaagagtacaatgaagaaataaaagaaaaacatatgaaaataaataagatctaataattgactgcattgcttttaatccaagaagtctatcatagtttttctttcctttttatatcagctggggaaaataaaattagtgcaatgttgcaaattgtaaatgcagtacggcaacctccacgccttagcagtacatgaacctctaacagatccatctggagtttactgctgttggtaacttctgttgcccggcagcgctgtgatcctacacatggatacccttcactgcctgtttgatactttccagtagagctttgcattccggggaatagtcccgttccagattgctgtacatatctgtgagtgtatttacatatgcttcaaaattctgctcactgataggtcccatctgtggaagctggatgtcagcaaggcttgaaatgagagcttggcttagacctgccagctctttcagcagactttcattgttctgttctatgagtttgttctcctcctctatcgtctttaagttgctctccatagatgtgatctgggtctgaagtttcatcatatctgcttcaattttaaggttggattcattcagttcctttatttcttcatccaaatgcctaatttcttcatcactctctattcccccagttgctttgagcttgatggtcatgagttcttcagaaaccttgccctttttgataacttgtgcattgagaggacatccagataagcttcggtgggtgacaaaaacattatttacatggcccagcccattgcagcctggcaagggacaatgtggtagctcttgtttgttcagtttccaggagagggaggctccattgagaggattctccttctgtctcttggcagccagaggacagccagaagctgtgcggtgtgatgtgtatttacctgatatgtgaccttggccatcacaccctatcacaggacatttcagttcagggtcttctttttcttccttggtaggggtcattttgacaccacctttccttgcacgagggcatccggacaagcttctgtgggaagcatagtttccagtcacgtgccccgagccatcgcagcctggggttggacacttaagctcctgagagttggcagccatgagggattttagagtcttatctgctaaaggacatccagaaacactgcgatgagatgcatagtttcctgtcacgtggccacttccatcacatcctggtgttggacaggtgattagttcctttttgagatctcttgcatgaagcttgggtttagggcttggtatagaggcctctccaggaaactttttttcctctaaattttctagagagctcactgggtctttctctttctcctcctctgtcttcccgtgagttttgctatagttgataggagtgtcccagccctcttggtcacaaagagcctgatagaatgctgcattgaccagaatgctgcttgttttgaatggggaagaggaaggagttggaatagaagtgttagaggaagttaggggtgcagacttgtccaggattcgattttttttcatgcttaagtccaatgtgccattttcatccacttctatttcggctcccttggcatgcagactctgtggcttgttggagaggatgtctgtggcttccctgcagcgggtggaaaggttcaggatggcagcagctgctgctatgtgggtgtcttcactacattgaccgtagctataagagctggcacggccagggctctgggtgtgggcgcctgcactaggcagtcgattaggaaatttcactggatttggaaaatgctttgattcaggaaatggtggtgtttttcgtccttgcactgtttgtatgagagggcgtttaccgaaaacttgggcatcaaaactggcataatcaaatggtacttttccaaacttctcttgttcttttgacactgtggctctgggagaggtgatggcttgtgacgggaaattgaattcaatttgcttcaccaaacttgtcctgtgggcctggtcaggacactgcccagtttggggagaatcaagctgatttttatcctgggacattgccaatttttcagctgcagcaattggacaaccagaaagactcctgtgggtgttgcggttgctgttcacatgaccccttcctgtgcatcccggcgtgggacacttgagcacattttcatgcatggcaagaatttccaggggaacccgcactttgtgggggcaccccgaaaggctgcggtggtgcgggtagagccctgtcacgtgtcccgtgccatcacatccagggatcgggcacttggtctccctcttttcaggccttggtgaatgtttattgttaaagatttgtcttccacccatgtcgataactttggtttgcctcctttcccctgctaggtgctccagcaggaacctatccagctctttgtaggtgttatggaaaacacaacctcgctcagcctgcagagcaattgcctgctccagcaaacttaaattccccttggccttttccaggtcactaccctcttccgtcattactgccaggctctcgctatcttcctcctcaacgtcagggaatgagggctgggcattgccatccaggggttctgcgagagcattctgcgggtctttcctttctgtttcagaatcacacctgttctcacaagggataaatttgtcaccttcagtttttatttcaggaacttccaataggtcttttttatgatctgttaaaacatactttgggactctaggtggtttggtttcttctgagaagttggagccactgtcccagccattttctgcactttcagagttactttcattgtcatcagaggagcagaagggtggctgagaatcatcaatcttgtctcttccatcatcagaatgaatcagaaagcactcgtctgcttcatcgctctctgcttttaaagactggatgccactgtcatttaaattttcacttacagtctgaacagatacatttttttcaaatttccccaagtgcattaaagacttgaccatgagctcttgataacaagagtatctgtcttccttcctactggagttttcttgtgcagttgaaagaagactttcatccataggttttatcatgatttcctctgcggtagagtgaccatgtgtttccaaggggccatcgtcctctgtcctgtcactgcggtcttcttggcagtctgcttttgggctgtagtgtcggggcttcattagcagggatttccttttgttgactggaacccccaaagcctgatcttcagctgttctcttctttgccatggagcaatcataggcaacactgagctcctggattagtgaatccattggcacctcggttcctttagagcgagtacgcagcgttttatcttcagcctctgcatccatctctctttttctccaggtaacttgtatgtcaactcagtttgccctgctgtgtcagggggactaaataaatgactttgtcttatttagtgataaatcctgaaattcattctttcttgcagaaaatttctaccgtcctgccttctctaccctttgcagtatatcaaagtgctcagctttttaatcatagatttctgtgtttcttgtaggatttgaccagacattaaatagatgcttcttcaacttaagtcagcaactgtagttccttccctaaaagctactggatctgaactggagagtttccatcactccttagtcttgatatgagcacgcagacacataaaatggaattgtcacaatgcttcagggacactcacaaaattgggggctttttttgtttgtttccaaaacttatatttctctcctccctggtgggctgaacggaaacactaaagctgtttctttgaaaggtagttcccatgatatgac

SEQ ID NO: 18691 - RNA, 4867 nt, Homo sapiens
  source 1..4867: mol_type = other RNA
tgagtgtgtgtgtgtgagtgtgtgtgtatattttgtagcatttgaagttttgtggcaagatttctatcaaattgaatgttgtcttgtttcctatggtgggtgagacccaaggtgccagtgtttgaagtaatcattcagattggagtagcattttttcatgtgttactatattttccattcctttccagtcaacccagtaagataaatgctatttcaggggatatggtatctacaaaatttttcatttggatgtgtttgtatttgctaagtacaaatctacaccaatattgtcacttgtatattgtaccaacatatggcaggaaagcctggctggtcacaccaagtcttatttttcatcttgggatacgagttgccaacgatctgatatgacttgaaaaacaaacagacaaatctgcatcactaaaaaggcttatgtttctttaaaacatttcaaataaataattcatattaacgaaaaccgtccagccaagtcgaatactttgctgattgctatatttaattattgctaacaaattctgagcaggctgttttccagcatcctgtgcttttgtgagtgcggattccccactagtgggcgccatttgtcttcttattccttccgtgcagctcaccttaccgcaaattcatttataaatacaaaaatcagtgaaaggtgggggaagaagtgtgcaataaaaatcaaactcaactatagtgcagtccttagacaaggatttccttcaccctttcctgtttcctcattaaaacccagcaagaaagatgacttgagaatagcatttctatttaaatcctattggaaaataaattaataaacacacttgtaaaaatacggcagacttcaaaatgcagttaaaagataaaaaactctttgattagtaataaataaattataaaaatgtcacatttattttacatatactttacaaaaaaaaaaagagtacaatgaagaaataaaagaaaaacatatgaaaataaataagatctaataattgactgcattgcttttaatccaagaagtctatcatagtttttctttcctttttatatcagctggggaaaataaaattagtgcaatgttgcaaattgtaaatgcagtacggcaacctccacgccttagcagtacatgaacctctaacagatccatctggagtttactgctgttggtaacttctgttgcccggcagcgctgtgatcctacacatggatacccttcactgcctgtttgatactttccagtagagctttgcattccggggaatagtcccgttccagattgctgtacatatctgtgagtgtatttacatatgcttcaaaattctgctcactgataggtcccatctgtggaagctggatgtcagcaaggcttgaaatgagagcttggcttagacctgccagctctttcagcagactttcattgttctgttctatgagtttgttctcctcctctatcgtctttaagttgctctccatagatgtgatctgggtctgaagtttcatcatatctgcttcaattttaaggttggattcattcagttcctttatttcttcatccaaatgcctaatttcttcatcactctctattcccccagttgctttgagcttgatggtcatgagttcttcagaaaccttgccctttttgataacttgtgcattgagaggacatccagataagcttcggtgggtgacaaaaacattatttacatggcccagcccattgcagcctggcaagggacaatgtggtagctcttgtttgttcagtttccaggagagggaggctccattgagaggattctccttctgtctcttggcagccagaggacagccagaagctgtgcggtgtgatgtgtatttacctgatatgtgaccttggccatcacaccctatcacaggacatttcagttcagggtcttctttttcttccttggtaggggtcattttgacaccacctttccttgcacgagggcatccggacaagcttctgtgggaagcatagtttccagtcacgtgccccgagccatcgcagcctggggttggacacttaagctcctgagagttggcagccatgagggattttagagtcttatctgctaaaggacatccagaaacactgcgatgagatgcatagtttcctgtcacgtggccacttccatcacatcctggtgttggacaggtgattagttcctttttgagatctcttgcatgaagcttgggtttagggcttggtatagaggcctctccaggaaactttttttcctctaaattttctagagagctcactgggtctttctctttctcctcctctgtcttcccgtgagttttgctatagttgataggagtgtcccagccctcttggtcacaaagagcctgatagaatgctgcattgaccagaatgctgcttgttttgaatggggaagaggaaggagttggaatagaagtgttagaggaagttaggggtgcagacttgtccaggattcgattttttttcatgcttaagtccaatgtgccattttcatccacttctatttcggctcccttggcatgcagactctgtggcttgttggagaggatgtctgtggcttccctgcagcgggtggaaaggttcaggatggcagcagctgctgctatgtgggtgtcttcactacattgaccgtagctataagagctggcacggccagggctctgggtgtgggcgcctgcactaggcagtcgattaggaaatttcactggatttggaaaatgctttgattcaggaaatggtggtgtttttcgtccttgcactgtttgtatgagagggcgtttaccgaaaacttgggcatcaaaactggcataatcaaatggtacttttccaaacttctcttgttcttttgacactgtggctctgggagaggtgatggcttgtgacgggaaattgaattcaatttgcttcaccaaacttgtcctgtgggcctggtcaggacactgcccagtttggggagaatcaagctgatttttatcctgggacattgccaatttttcagctgcagcaattggacaaccagaaagactcctgtgggtgttgcggttgctgttcacatgaccccttcctgtgcatcccggcgtgggacacttgagcacattttcatgcatggcaagaatttccaggggaacccgcactttgtgggggcaccccgaaaggctgcggtggtgcgggtagagccctgtcacgtgtcccgtgccatcacatccagggatcgggcacttggtctccctcttttcaggccttggtgaatgtttattgttaaagatttgtcttccacccatgtcgataactttggtttgcctcctttcccctgctaggtgctccagcaggaacctatccagctctttgtaggtgttatggaaaacacaacctcgctcagcctgcagagcaattgcctgctccagcaaacttaaattccccttggccttttccaggtcactaccctcttccgtcattactgccaggctctcgctatcttcctcctcaacgtcagggaatgagggctgggcattgccatccaggggttctgcgagagcattctgcgggtctttcctttctgtttcagaatcacacctgttctcacaagggataaatttgtcaccttcagtttttatttcaggaacttccaataggtcttttttatgatctgttaaaacatactttgggactctaggtggtttggtttcttctgagaagttggagccactgtcccagccattttctgcactttcagagttactttcattgtcatcagaggagcagaagggtggctgagaatcatcaatcttgtctcttccatcatcagaatgaatcagaaagcactcgtctgcttcatcgctctctgcttttaaagactggatgccactgtcatttaaattttcacttacagtctgaacagatacatttttttcaaatttccccaagtgcattaaagacttgaccatgagctcttgataacaagagtatctgtcttccttcctactggagttttcttgtgcagttgaaagaagactttcatccataggttttatcatgatttcctctgcggtagagtgaccatgtgtttccaaggggccatcgtcctctgtcctgtcactgcggtcttcttggcagtctgcttttgggctgtagtgtcggggcttcattagcagggatttccttttgttgactggaacccccaaagcctgatcttcagctgttctcttctttgccatggagcaatcataggcaacactgagctcctggattagtgaatccattggcacctcggttcctttagagcgagtacgcagcgttttatcttcagcctctgcatccatctctctttttctccaggtaacttgtatgtcaactcagtttgccctgctgtgtcagggggactaaataaatgactttgtcttatttagtgataaatcctgaaattcattctttcttgcagaaaatttctaccgtcctgccttctctaccctttgcagtatatcaaagtgctcagctttttaatcatagatttctgtgtttcttgtaggatttgaccagacattaaatagatgcttcttcaacttaagtcagcaactgtagttccttccctaaaagctactggatctgaactggagagtttccatcactcctttacctggcgaacgtctacaggtgtgtcgaaagttatcttttcctggatgtgttccaaaatgctcttatgctatttctcttaggatttctccacgctgccccattcagaaattttattattttctctagtattcccctgaggtcacattcagttaaaaacatcctgcccttctccctacaaaaaggttccatagaatc

SEQ ID NO: 18692 - RNA, 5001 nt, Homo sapiens
  source 1..5001: mol_type = other RNA
tgagtgtgtgtgtgtgagtgtgtgtgtatattttgtagcatttgaagttttgtggcaagatttctatcaaattgaatgttgtcttgtttcctatggtgggtgagacccaaggtgccagtgtttgaagtaatcattcagattggagtagcattttttcatgtgttactatattttccattcctttccagtcaacccagtaagataaatgctatttcaggggatatggtatctacaaaatttttcatttggatgtgtttgtatttgctaagtacaaatctacaccaatattgtcacttgtatattgtaccaacatatggcaggaaagcctggctggtcacaccaagtcttatttttcatcttgggatacgagttgccaacgatctgatatgacttgaaaaacaaacagacaaatctgcatcactaaaaaggcttatgtttctttaaaacatttcaaataaataattcatattaacgaaaaccgtccagccaagtcgaatactttgctgattgctatatttaattattgctaacaaattctgagcaggctgttttccagcatcctgtgcttttgtgagtgcggattccccactagtgggcgccatttgtcttcttattccttccgtgcagctcaccttaccgcaaattcatttataaatacaaaaatcagtgaaaggtgggggaagaagtgtgcaataaaaatcaaactcaactatagtgcagtccttagacaaggatttccttcaccctttcctgtttcctcattaaaacccagcaagaaagatgacttgagaatagcatttctatttaaatcctattggaaaataaattaataaacacacttgtaaaaatacggcagacttcaaaatgcagttaaaagataaaaaactctttgattagtaataaataaattataaaaatgtcacatttattttacatatactttacaaaaaaaaaaagagtacaatgaagaaataaaagaaaaacatatgaaaataaataagatctaataattgactgcattgcttttaatccaagaagtctatcatagtttttctttcctttttatatcagctggggaaaataaaattagtgcaatgttgcaaattgtaaatgcagtacggcaacctccacgccttagcagtacatgaacctctaacagatccatctggagtttactgctgttggtaacttctgttgcccggcagcgctgtgatcctacacatggatacccttcactgcctgtttgatactttccagtagagctttgcattccggggaatagtcccgttccagattgctgtacatatctgtgagtgtatttacatatgcttcaaaattctgctcactgataggtcccatctgtggaagctggatgtcagcaaggcttgaaatgagagcttggcttagacctgccagctctttcagcagactttcattgttctgttctatgagtttgttctcctcctctatcgtctttaagttgctctccatagatgtgatctgggtctgaagtttcatcatatctgcttcaattttaaggttggattcattcagttcctttatttcttcatccaaatgcctaatttcttcatcactctctattcccccagttgctttgagcttgatggtcatgagttcttcagaaaccttgccctttttgataacttgtgcattgagaggacatccagataagcttcggtgggtgacaaaaacattatttacatggcccagcccattgcagcctggcaagggacaatgtggtagctcttgtttgttcagtttccaggagagggaggctccattgagaggattctccttctgtctcttggcagccagaggacagccagaagctgtgcggtgtgatgtgtatttacctgatatgtgaccttggccatcacaccctatcacaggacatttcagttcagggtcttctttttcttccttggtaggggtcattttgacaccacctttccttgcacgagggcatccggacaagcttctgtgggaagcatagtttccagtcacgtgccccgagccatcgcagcctggggttggacacttaagctcctgagagttggcagccatgagggattttagagtcttatctgctaaaggacatccagaaacactgcgatgagatgcatagtttcctgtcacgtggccacttccatcacatcctggtgttggacaggtgattagttcctttttgagatctcttgcatgaagcttgggtttagggcttggtatagaggcctctccaggaaactttttttcctctaaattttctagagagctcactgggtctttctctttctcctcctctgtcttcccgtgagttttgctatagttgataggagtgtcccagccctcttggtcacaaagagcctgatagaatgctgcattgaccagaatgctgcttgttttgaatggggaagaggaaggagttggaatagaagtgttagaggaagttaggggtgcagacttgtccaggattcgattttttttcatgcttaagtccaatgtgccattttcatccacttctatttcggctcccttggcatgcagactctgtggcttgttggagaggatgtctgtggcttccctgcagcgggtggaaaggttcaggatggcagcagctgctgctatgtgggtgtcttcactacattgaccgtagctataagagctggcacggccagggctctgggtgtgggcgcctgcactaggcagtcgattaggaaatttcactggatttggaaaatgctttgattcaggaaatggtggtgtttttcgtccttgcactgtttgtatgagagggcgtttaccgaaaacttgggcatcaaaactggcataatcaaatggtacttttccaaacttctcttgttcttttgacactgtggctctgggagaggtgatggcttgtgacgggaaattgaattcaatttgcttcaccaaacttgtcctgtgggcctggtcaggacactgcccagtttggggagaatcaagctgatttttatcctgggacattgccaatttttcagctgcagcaattggacaaccagaaagactcctgtgggtgttgcggttgctgttcacatgaccccttcctgtgcatcccggcgtgggacacttgagcacattttcatgcatggcaagaatttccaggggaacccgcactttgtgggggcaccccgaaaggctgcggtggtgcgggtagagccctgtcacgtgtcccgtgccatcacatccagggatcgggcacttggtctccctcttttcaggccttggtgaatgtttattgttaaagatttgtcttccacccatgtcgataactttggtttgcctcctttcccctgctaggtgctccagcaggaacctatccagctctttgtaggtgttatggaaaacacaacctcgctcagcctgcagagcaattgcctgctccagcaaacttaaattccccttggccttttccaggtcactaccctcttccgtcattactgccaggctctcgctatcttcctcctcaacgtcagggaatgagggctgggcattgccatccaggggttctgcgagagcattctgcgggtctttcctttctgtttcagaatcacacctgttctcacaagggataaatttgtcaccttcagtttttatttcaggaacttccaataggtcttttttatgatctgttaaaacatactttgggactctaggtggtttggtttcttctgagaagttggagccactgtcccagccattttctgcactttcagagttactttcattgtcatcagaggagcagaagggtggctgagaatcatcaatcttgtctcttccatcatcagaatgaatcagaaagcactcgtctgcttcatcgctctctgcttttaaagactggatgccactgtcatttaaattttcacttacagtctgaacagatacatttttttcaaatttccccaagtgcattaaagacttgaccatgagctcttgataacaagagtatctgtcttccttcctactggagttttcttgtgcagttgaaagaagactttcatccataggttttatcatgatttcctctgcggtagagtgaccatgtgtttccaaggggccatcgtcctctgtcctgtcactgcggtcttcttggcagtctgcttttgggctgtagtgtcggggcttcattagcagggatttccttttgttgactggaacccccaaagcctgatcttcagctgttctcttctttgccatggagcaatcataggcaacactgagctcctggattagtgaatccattggcacctcggttcctttagagcgagtacgcagcgttttatcttcagcctctgcatccatctctctttttctccaggtaacttgtatgtcaactcagtttgccctgctgtgtcagggggactaaataaatgactttgtcttatttagtgataaatcctgaaattcattctttcttgcagaaaatttctaccgtcctgccttctctaccctttgcagtatatcaaagtgctcagctttttaatcatagatttctgtgtttcttgtaggatttgaccagacattaaatagatgcttcttcaacttaagtcagcaactgtagttccttccctaaaagctactggatctgaactggagagtttccatcactcctttacctggcgaacgtctacaggtgtgtcgaaagttatcttttcctggatgtgttccaaaatgctcttatgctatttctcttaggatttctccacgctgccccattcagaaattttattattttcttccacaactctgccaggcactggtttttgcgtgggatgatgccagcttctctcttcatgtggccttattaaaagccatggtttccgagatgtaaaacacccacagttacctcaattatttttctctccttacctctagtattcccctgaggtcacattcagttaaaaacatcctgcccttctccctacaaaaaggttccatagaatc

SEQ ID NO: 18693 - RNA, 4766 nt, Homo sapiens
  source 1..4766: mol_type = other RNA
tgagtgtgtgtgtgtgagtgtgtgtgtatattttgtagcatttgaagttttgtggcaagatttctatcaaattgaatgttgtcttgtttcctatggtgggtgagacccaaggtgccagtgtttgaagtaatcattcagattggagtagcattttttcatgtgttactatattttccattcctttccagtcaacccagtaagataaatgctatttcaggggatatggtatctacaaaatttttcatttggatgtgtttgtatttgctaagtacaaatctacaccaatattgtcacttgtatattgtaccaacatatggcaggaaagcctggctggtcacaccaagtcttatttttcatcttgggatacgagttgccaacgatctgatatgacttgaaaaacaaacagacaaatctgcatcactaaaaaggcttatgtttctttaaaacatttcaaataaataattcatattaacgaaaaccgtccagccaagtcgaatactttgctgattgctatatttaattattgctaacaaattctgagcaggctgttttccagcatcctgtgcttttgtgagtgcggattccccactagtgggcgccatttgtcttcttattccttccgtgcagctcaccttaccgcaaattcatttataaatacaaaaatcagtgaaaggtgggggaagaagtgtgcaataaaaatcaaactcaactatagtgcagtccttagacaaggatttccttcaccctttcctgtttcctcattaaaacccagcaagaaagatgacttgagaatagcatttctatttaaatcctattggaaaataaattaataaacacacttgtaaaaatacggcagacttcaaaatgcagttaaaagataaaaaactctttgattagtaataaataaattataaaaatgtcacatttattttacatatactttacaaaaaaaaaaagagtacaatgaagaaataaaagaaaaacatatgaaaataaataagatctaataattgactgcattgcttttaatccaagaagtctatcatagtttttctttcctttttatatcagctggggaaaataaaattagtgcaatgttgcaaattgtaaatgcagtacggcaacctccacgccttagcagtacatgaacctctaacagatccatctggagtttactgctgttggtaacttctgttgcccggcagcgctgtgatcctacacatggatacccttcactgcctgtttgatactttccagtagagctttgcattccggggaatagtcccgttccagattgctgtacatatctgtgagtgtatttacatatgcttcaaaattctgctcactgataggtcccatctgtggaagctggatgtcagcaaggcttgaaatgagagcttggcttagacctgccagctctttcagcagactttcattgttctgttctatgagtttgttctcctcctctatcgtctttaagttgctctccatagatgtgatctgggtctgaagtttcatcatatctgcttcaattttaaggttggattcattcagttcctttatttcttcatccaaatgcctaatttcttcatcactctctattcccccagttgctttgagcttgatggtcatgagttcttcagaaaccttgccctttttgataacttgtgcattgagaggacatccagataagcttcggtgggtgacaaaaacattatttacatggcccagcccattgcagcctggcaagggacaatgtggtagctcttgtttgttcagtttccaggagagggaggctccattgagaggattctccttctgtctcttggcagccagaggacagccagaagctgtgcggtgtgatgtgtatttacctgatatgtgaccttggccatcacaccctatcacaggacatttcagttcagggtcttctttttcttccttggtaggggtcattttgacaccacctttccttgcacgagggcatccggacaagcttctgtgggaagcatagtttccagtcacgtgccccgagccatcgcagcctggggttggacacttaagctcctgagagttggcagccatgagggattttagagtcttatctgctaaaggacatccagaaacactgcgatgagatgcatagtttcctgtcacgtggccacttccatcacatcctggtgttggacaggtgattagttcctttttgagatctcttgcatgaagcttgggtttagggcttggtatagaggcctctccaggaaactttttttcctctaaattttctagagagctcactgggtctttctctttctcctcctctgtcttcccgtgagttttgctatagttgataggagtgtcccagccctcttggtcacaaagagcctgatagaatgctgcattgaccagaatgctgcttgttttgaatggggaagaggaaggagttggaatagaagtgttagaggaagttaggggtgcagacttgtccaggattcgattttttttcatgcttaagtccaatgtgccattttcatccacttctatttcggctcccttggcatgcagactctgtggcttgttggagaggatgtctgtggcttccctgcagcgggtggaaaggttcaggatggcagcagctgctgctatgtgggtgtcttcactacattgaccgtagctataagagctggcacggccagggctctgggtgtgggcgcctgcactaggcagtcgattaggaaatttcactggatttggaaaatgctttgattcaggaaatggtggtgtttttcgtccttgcactgtttgtatgagagggcgtttaccgaaaacttgggcatcaaaactggcataatcaaatggtacttttccaaacttctcttgttcttttgacactgtggctctgggagaggtgatggcttgtgacgggaaattgaattcaatttgcttcaccaaacttgtcctgtgggcctggtcaggacactgcccagtttggggagaatcaagctgatttttatcctgggacattgccaatttttcagctgcagcaattggacaaccagaaagactcctgtgggtgttgcggttgctgttcacatgaccccttcctgtgcatcccggcgtgggacacttgagcacattttcatgcatggcaagaatttccaggggaacccgcactttgtgggggcaccccgaaaggctgcggtggtgcgggtagagccctgtcacgtgtcccgtgccatcacatccagggatcgggcacttggtctccctcttttcaggccttggtgaatgtttattgttaaagatttgtcttccacccatgtcgataactttggtttgcctcctttcccctgctaggtgctccagcaggaacctatccagctctttgtaggtgttatggaaaacacaacctcgctcagcctgcagagcaattgcctgctccagcaaacttaaattccccttggccttttccaggtcactaccctcttccgtcattactgccaggctctcgctatcttcctcctcaacgtcagggaatgagggctgggcattgccatccaggggttctgcgagagcattctgcgggtctttcctttctgtttcagaatcacacctgttctcacaagggataaatttgtcaccttcagtttttatttcaggaacttccaataggtcttttttatgatctgttaaaacatactttgggactctaggtggtttggtttcttctgagaagttggagccactgtcccagccattttctgcactttcagagttactttcattgtcatcagaggagcagaagggtggctgagaatcatcaatcttgtctcttccatcatcagaatgaatcagaaagcactcgtctgcttcatcgctctctgcttttaaagactggatgccactgtcatttaaattttcacttacagtctgaacagatacatttttttcaaatttccccaagtgcattaaagacttgaccatgagctcttgataacaagagtatctgtcttccttcctactggagttttcttgtgcagttgaaagaagactttcatccataggttttatcatgatttcctctgcggtagagtgaccatgtgtttccaaggggccatcgtcctctgtcctgtcactgcggtcttcttggcagtctgcttttgggctgtagtgtcggggcttcattagcagggatttccttttgttgactggaacccccaaagcctgatcttcagctgttctcttctttgccatggagcaatcataggcaacactgagctcctggattagtgaatccattggcacctcggttcctttagagcgagtacgcagcgttttatcttcagcctctgcatccatctctctttttctccaggtaacttgtatgtcaactcagtttgccctgctgtgtcagggggactaaataaatgactttgtcttatttagtgataaatcctgaaattcattctttcttgcagaaaatttctaccgtcctgccttctctaccctttgcagtatatcaaagtgctcagctttttaatcatagatttctgtgtttcttgtaggatttgaccagacattaaatagatgcttcttcaacttaagtcagcaactgtagttccttccctaaaagctactggatctgaactggagagtttccatcactcttttttgtttgtttccaaaacttatatttctctcctccctggtgggctgaacggaaacactaaagctgtttctttgaaaggtagttcccatgatatgac

SEQ ID NO: 18694 - RNA, 4955 nt, Homo sapiens
  source 1..4955: mol_type = other RNA
tgagtgtgtgtgtgtgagtgtgtgtgtatattttgtagcatttgaagttttgtggcaagatttctatcaaattgaatgttgtcttgtttcctatggtgggtgagacccaaggtgccagtgtttgaagtaatcattcagattggagtagcattttttcatgtgttactatattttccattcctttccagtcaacccagtaagataaatgctatttcaggggatatggtatctacaaaatttttcatttggatgtgtttgtatttgctaagtacaaatctacaccaatattgtcacttgtatattgtaccaacatatggcaggaaagcctggctggtcacaccaagtcttatttttcatcttgggatacgagttgccaacgatctgatatgacttgaaaaacaaacagacaaatctgcatcactaaaaaggcttatgtttctttaaaacatttcaaataaataattcatattaacgaaaaccgtccagccaagtcgaatactttgctgattgctatatttaattattgctaacaaattctgagcaggctgttttccagcatcctgtgcttttgtgagtgcggattccccactagtgggcgccatttgtcttcttattccttccgtgcagctcaccttaccgcaaattcatttataaatacaaaaatcagtgaaaggtgggggaagaagtgtgcaataaaaatcaaactcaactatagtgcagtccttagacaaggatttccttcaccctttcctgtttcctcattaaaacccagcaagaaagatgacttgagaatagcatttctatttaaatcctattggaaaataaattaataaacacacttgtaaaaatacggcagacttcaaaatgcagttaaaagataaaaaactctttgattagtaataaataaattataaaaatgtcacatttattttacatatactttacaaaaaaaaaaagagtacaatgaagaaataaaagaaaaacatatgaaaataaataagatctaataattgactgcattgcttttaatccaagaagtctatcatagtttttctttcctttttatatcagctggggaaaataaaattagtgcaatgttgcaaattgtaaatgcagtacggcaacctccacgccttagcagtacatgaacctctaacagatccatctggagtttactgctgttggtaacttctgttgcccggcagcgctgtgatcctacacatggatacccttcactgcctgtttgatactttccagtagagctttgcattccggggaatagtcccgttccagattgctgtacatatctgtgagtgtatttacatatgcttcaaaattctgctcactgataggtcccatctgtggaagctggatgtcagcaaggcttgaaatgagagcttggcttagacctgccagctctttcagcagactttcattgttctgttctatgagtttgttctcctcctctatcgtctttaagttgctctccatagatgtgatctgggtctgaagtttcatcatatctgcttcaattttaaggttggattcattcagttcctttatttcttcatccaaatgcctaatttcttcatcactctctattcccccagttgctttgagcttgatggtcatgagttcttcagaaaccttgccctttttgataacttgtgcattgagaggacatccagataagcttcggtgggtgacaaaaacattatttacatggcccagcccattgcagcctggcaagggacaatgtggtagctcttgtttgttcagtttccaggagagggaggctccattgagaggattctccttctgtctcttggcagccagaggacagccagaagctgtgcggtgtgatgtgtatttacctgatatgtgaccttggccatcacaccctatcacaggacatttcagttcagggtcttctttttcttccttggtaggggtcattttgacaccacctttccttgcacgagggcatccggacaagcttctgtgggaagcatagtttccagtcacgtgccccgagccatcgcagcctggggttggacacttaagctcctgagagttggcagccatgagggattttagagtcttatctgctaaaggacatccagaaacactgcgatgagatgcatagtttcctgtcacgtggccacttccatcacatcctggtgttggacaggtgattagttcctttttgagatctcttgcatgaagcttgggtttagggcttggtatagaggcctctccaggaaactttttttcctctaaattttctagagagctcactgggtctttctctttctcctcctctgtcttcccgtgagttttgctatagttgataggagtgtcccagccctcttggtcacaaagagcctgatagaatgctgcattgaccagaatgctgcttgttttgaatggggaagaggaaggagttggaatagaagtgttagaggaagttaggggtgcagacttgtccaggattcgattttttttcatgcttaagtccaatgtgccattttcatccacttctatttcggctcccttggcatgcagactctgtggcttgttggagaggatgtctgtggcttccctgcagcgggtggaaaggttcaggatggcagcagctgctgctatgtgggtgtcttcactacattgaccgtagctataagagctggcacggccagggctctgggtgtgggcgcctgcactaggcagtcgattaggaaatttcactggatttggaaaatgctttgattcaggaaatggtggtgtttttcgtccttgcactgtttgtatgagagggcgtttaccgaaaacttgggcatcaaaactggcataatcaaatggtacttttccaaacttctcttgttcttttgacactgtggctctgggagaggtgatggcttgtgacgggaaattgaattcaatttgcttcaccaaacttgtcctgtgggcctggtcaggacactgcccagtttggggagaatcaagctgatttttatcctgggacattgccaatttttcagctgcagcaattggacaaccagaaagactcctgtgggtgttgcggttgctgttcacatgaccccttcctgtgcatcccggcgtgggacacttgagcacattttcatgcatggcaagaatttccaggggaacccgcactttgtgggggcaccccgaaaggctgcggtggtgcgggtagagccctgtcacgtgtcccgtgccatcacatccagggatcgggcacttggtctccctcttttcaggccttggtgaatgtttattgttaaagatttgtcttccacccatgtcgataactttggtttgcctcctttcccctgctaggtgctccagcaggaacctatccagctctttgtaggtgttatggaaaacacaacctcgctcagcctgcagagcaattgcctgctccagcaaacttaaattccccttggccttttccaggtcactaccctcttccgtcattactgccaggctctcgctatcttcctcctcaacgtcagggaatgagggctgggcattgccatccaggggttctgcgagagcattctgcgggtctttcctttctgtttcagaatcacacctgttctcacaagggataaatttgtcaccttcagtttttatttcaggaacttccaataggtcttttttatgatctgttaaaacatactttgggactctaggtggtttggtttcttctgagaagttggagccactgtcccagccattttctgcactttcagagttactttcattgtcatcagaggagcagaagggtggctgagaatcatcaatcttgtctcttccatcatcagaatgaatcagaaagcactcgtctgcttcatcgctctctgcttttaaagactggatgccactgtcatttaaattttcacttacagtctgaacagatacatttttttcaaatttccccaagtgcattaaagacttgaccatgagctcttgataacaagagtatctgtcttccttcctactggagttttcttgtgcagttgaaagaagactttcatccataggttttatcatgatttcctctgcggtagagtgaccatgtgtttccaaggggccatcgtcctctgtcctgtcactgcggtcttcttggcagtctgcttttgggctgtagtgtcggggcttcattagcagggatttccttttgttgactggaacccccaaagcctgatcttcagctgttctcttctttgccatggagcaatcataggcaacactgagctcctggattagtgaatccattggcacctcggttcctttagagcgagtacgcagcgttttatcttcagcctctgcatccatctctctttttctccaggtaacttgtatgtcaactcagtttgccctgctgtgtcagggggactaaataaatgactttgtcttatttagtgataaatcctgaaattcattctttcttgcagaaaatttctaccgtcctgccttctctaccctttgcagtatatcaaagtgctcagctttttaatcatagatttctgtgtttcttgtaggatttgaccagacattaaatagatgcttcttcaacttaagtcagcaactgtagttcctttacctggcgaacgtctacaggtgtgtcgaaagttatcttttcctggatgtgttccaaaatgctcttatgctatttctcttaggatttctccacgctgccccattcagaaattttattattttcttccacaactctgccaggcactggtttttgcgtgggatgatgccagcttctctcttcatgtggccttattaaaagccatggtttccgagatgtaaaacacccacagttacctcaattatttttctctccttacctctagtattcccctgaggtcacattcagttaaaaacatcctgcccttctccctacaaaaaggttccatagaatc

SEQ ID NO: 18695 - RNA, 4535 nt, Homo sapiens
  source 1..4535: mol_type = other RNA
tgagtgtgtgtgtgtgagtgtgtgtgtatattttgtagcatttgaagttttgtggcaagatttctatcaaattgaatgttgtcttgtttcctatggtgggtgagacccaaggtgccagtgtttgaagtaatcattcagattggagtagcattttttcatgtgttactatattttccattcctttccagtcaacccagtaagataaatgctatttcaggggatatggtatctacaaaatttttcatttggatgtgtttgtatttgctaagtacaaatctacaccaatattgtcacttgtatattgtaccaacatatggcaggaaagcctggctggtcacaccaagtcttatttttcatcttgggatacgagttgccaacgatctgatatgacttgaaaaacaaacagacaaatctgcatcactaaaaaggcttatgtttctttaaaacatttcaaataaataattcatattaacgaaaaccgtccagccaagtcgaatactttgctgattgctatatttaattattgctaacaaattctgagcaggctgttttccagcatcctgtgcttttgtgagtgcggattccccactagtgggcgccatttgtcttcttattccttccgtgcagctcaccttaccgcaaattcatttataaatacaaaaatcagtgaaaggtgggggaagaagtgtgcaataaaaatcaaactcaactatagtgcagtccttagacaaggatttccttcaccctttcctgtttcctcattaaaacccagcaagaaagatgacttgagaatagcatttctatttaaatcctattggaaaataaattaataaacacacttgtaaaaatacggcagacttcaaaatgcagttaaaagataaaaaactctttgattagtaataaataaattataaaaatgtcacatttattttacatatactttacaaaaaaaaaaagagtacaatgaagaaataaaagaaaaacatatgaaaataaataagatctaataattgactgcattgcttttaatccaagaagtctatcatagtttttctttcctttttatatcagctggggaaaataaaattagtgcaatgttgcaaattgtaaatgcagtacggcaacctccacgccttagcagtacatgaacctctaacagatccatctggagtttactgctgttggtaacttctgttgcccggcagcgctgtgatcctacacatggatacccttcactgcctgtttgatactttccagtagagctttgcattccggggaatagtcccgttccagattgctgtacatatctgtgagtgtatttacatatgcttcaaaattctgctcactgataggtcccatctgtggaagctggatgtcagcaaggcttgaaatgagagcttggcttagacctgccagctctttcagcagactttcattgttctgttctatgagtttgttctcctcctctatcgtctttaagttgctctccatagatgtgatctgggtctgaagtttcatcatatctgcttcaattttaaggttggattcattcagttcctttatttcttcatccaaatgcctaatttcttcatcactctctattcccccagttgctttgagcttgatggtcatgagttcttcagaaaccttgccctttttgataacttgtgcattgagaggacatccagataagcttcggtgggtgacaaaaacattatttacatggcccagcccattgcagcctggcaagggacaatgtggtagctcttgtttgttcagtttccaggagagggaggctccattgagaggattctccttctgtctcttggcagccagaggacagccagaagctgtgcggtgtgatgtgtatttacctgatatgtgaccttggccatcacaccctatcacaggacatttcagttcagggtcttctttttcttccttggtaggggtcattttgacaccacctttccttgcacgagggcatccggacaagcttctgtgggaagcatagtttccagtcacgtgccccgagccatcgcagcctggggttggacacttaagctcctgagagttggcagccatgagggattttagagtcttatctgctaaaggacatccagaaacactgcgatgagatgcatagtttcctgtcacgtggccacttccatcacatcctggtgttggacaggtgattagttcctttttgagatctcttgcatgaagcttgggtttagggcttggtatagaggcctctccaggaaactttttttcctctaaattttctagagagctcactgggtctttctctttctcctcctctgtcttcccgtgagttttgctatagttgataggagtgtcccagccctcttggtcacaaagagcctgatagaatgctgcattgaccagaatgctgcttgttttgaatggggaagaggaaggagttggaatagaagtgttagaggaagttaggggtgcagacttgtccaggattcgattttttttcatgcttaagtccaatgtgccattttcatccacttctatttcggctcccttggcatgcagactctgtggcttgttggagaggatgtctgtggcttccctgcagcgggtggaaaggttcaggatggcagcagctgctgctatgtgggtgtcttcactacattgaccgtagctataagagctggcacggccagggctctgggtgtgggcgcctgcactaggcagtcgattaggaaatttcactggatttggaaaatgctttgattcaggaaatggtggtgtttttcgtccttgcactgtttgtatgagagggcgtttaccgaaaacttgggcatcaaaactggcataatcaaatggtacttttccaaacttctcttgttcttttgacactgtggctctgggagaggtgatggcttgtgacgggaaattgaattcaatttgcttcaccaaacttgtcctgtgggcctggtcaggacactgcccagtttggggagaatcaagctgatttttatcctgggacattgccaatttttcagctgcagcaattggacaaccagaaagactcctgtgggtgttgcggttgctgttcacatgaccccttcctgtgcatcccggcgtgggacacttgagcacattttcatgcatggcaagaatttccaggggaacccgcactttgtgggggcaccccgaaaggctgcggtggtgcgggtagagccctgtcacgtgtcccgtgccatcacatccagggatcgggcacttggtctccctcttttcaggccttggtgaatgtttattgttaaagatttgtcttccacccatgtcgataactttggtttgcctcctttcccctgctaggtgctccagcaggaacctatccagctctttgtaggtgttatggaaaacacaacctcgctcagcctgcagagcaattgcctgctccagcaaacttaaattccccttggccttttccaggtcactaccctcttccgtcattactgccaggctctcgctatcttcctcctcaacgtcagggaatgagggctgggcattgccatccaggggttctgcgagagcattctgcgggtctttcctttctgtttcagaatcacacctgttctcacaagggataaatttgtcaccttcagtttttatttcaggaacttccaataggtcttttttatgatctgttaaaacatactttgggactctaggtggtttggtttcttctgagaagttggagccactgtcccagccattttctgcactttcagagttactttcattgtcatcagaggagcagaagggtggctgagaatcatcaatcttgtctcttccatcatcagaatgaatcagaaagcactcgtctgcttcatcgctctctgcttttaaagactggatgccactgtcatttaaattttcacttacagtctgaacagatacatttttttcaaatttccccaagtgcattaaagacttgaccatgagctcttgataacaagagtatctgtcttccttcctactggagttttcttgtgcagttgaaagaagactttcatccataggttttatcatgatttcctctgcggtagagtgaccatgtgtttccaaggggccatcgtcctctgtcctgtcactgcggtcttcttggcagtctgcttttgggctgtagtgtcggggcttcattagcagggatttccttttgttgactggaacccccaaagcctgatcttcagctgttctcttctttgccatggagcaatcataggcaacactgagctcctggattagtgaatccattggcacctcggttcctttagagcgagtacgcagcgttttatcttcagcctctgcatccatcttccctaaaagctactggatctgaactggagagtttccatcactccggtgcctcctagcctttgttctgcctctcacgctgacatcagggaagcagtgatgtagaataaagcaggggtgggctaggttagtccagtgtttgtgtcgttgtgtggtgtgcagggacactctgtgat

SEQ ID NO: 18696 - RNA, 4614 nt, Homo sapiens
  source 1..4614: mol_type = other RNA
tgagtgtgtgtgtgtgagtgtgtgtgtatattttgtagcatttgaagttttgtggcaagatttctatcaaattgaatgttgtcttgtttcctatggtgggtgagacccaaggtgccagtgtttgaagtaatcattcagattggagtagcattttttcatgtgttactatattttccattcctttccagtcaacccagtaagataaatgctatttcaggggatatggtatctacaaaatttttcatttggatgtgtttgtatttgctaagtacaaatctacaccaatattgtcacttgtatattgtaccaacatatggcaggaaagcctggctggtcacaccaagtcttatttttcatcttgggatacgagttgccaacgatctgatatgacttgaaaaacaaacagacaaatctgcatcactaaaaaggcttatgtttctttaaaacatttcaaataaataattcatattaacgaaaaccgtccagccaagtcgaatactttgctgattgctatatttaattattgctaacaaattctgagcaggctgttttccagcatcctgtgcttttgtgagtgcggattccccactagtgggcgccatttgtcttcttattccttccgtgcagctcaccttaccgcaaattcatttataaatacaaaaatcagtgaaaggtgggggaagaagtgtgcaataaaaatcaaactcaactatagtgcagtccttagacaaggatttccttcaccctttcctgtttcctcattaaaacccagcaagaaagatgacttgagaatagcatttctatttaaatcctattggaaaataaattaataaacacacttgtaaaaatacggcagacttcaaaatgcagttaaaagataaaaaactctttgattagtaataaataaattataaaaatgtcacatttattttacatatactttacaaaaaaaaaaagagtacaatgaagaaataaaagaaaaacatatgaaaataaataagatctaataattgactgcattgcttttaatccaagaagtctatcatagtttttctttcctttttatatcagctggggaaaataaaattagtgcaatgttgcaaattgtaaatgcagtacggcaacctccacgccttagcagtacatgaacctctaacagatccatctggagtttactgctgttggtaacttctgttgcccggcagcgctgtgatcctacacatggatacccttcactgcctgtttgatactttccagtagagctttgcattccggggaatagtcccgttccagattgctgtacatatctgtgagtgtatttacatatgcttcaaaattctgctcactgataggtcccatctgtggaagctggatgtcagcaaggcttgaaatgagagcttggcttagacctgccagctctttcagcagactttcattgttctgttctatgagtttgttctcctcctctatcgtctttaagttgctctccatagatgtgatctgggtctgaagtttcatcatatctgcttcaattttaaggttggattcattcagttcctttatttcttcatccaaatgcctaatttcttcatcactctctattcccccagttgctttgagcttgatggtcatgagttcttcagaaaccttgccctttttgataacttgtgcattgagaggacatccagataagcttcggtgggtgacaaaaacattatttacatggcccagcccattgcagcctggcaagggacaatgtggtagctcttgtttgttcagtttccaggagagggaggctccattgagaggattctccttctgtctcttggcagccagaggacagccagaagctgtgcggtgtgatgtgtatttacctgatatgtgaccttggccatcacaccctatcacaggacatttcagttcagggtcttctttttcttccttggtaggggtcattttgacaccacctttccttgcacgagggcatccggacaagcttctgtgggaagcatagtttccagtcacgtgccccgagccatcgcagcctggggttggacacttaagctcctgagagttggcagccatgagggattttagagtcttatctgctaaaggacatccagaaacactgcgatgagatgcatagtttcctgtcacgtggccacttccatcacatcctggtgttggacaggtgattagttcctttttgagatctcttgcatgaagcttgggtttagggcttggtatagaggcctctccaggaaactttttttcctctaaattttctagagagctcactgggtctttctctttctcctcctctgtcttcccgtgagttttgctatagttgataggagtgtcccagccctcttggtcacaaagagcctgatagaatgctgcattgaccagaatgctgcttgttttgaatggggaagaggaaggagttggaatagaagtgttagaggaagttaggggtgcagacttgtccaggattcgattttttttcatgcttaagtccaatgtgccattttcatccacttctatttcggctcccttggcatgcagactctgtggcttgttggagaggatgtctgtggcttccctgcagcgggtggaaaggttcaggatggcagcagctgctgctatgtgggtgtcttcactacattgaccgtagctataagagctggcacggccagggctctgggtgtgggcgcctgcactaggcagtcgattaggaaatttcactggatttggaaaatgctttgattcaggaaatggtggtgtttttcgtccttgcactgtttgtatgagagggcgtttaccgaaaacttgggcatcaaaactggcataatcaaatggtacttttccaaacttctcttgttcttttgacactgtggctctgggagaggtgatggcttgtgacgggaaattgaattcaatttgcttcaccaaacttgtcctgtgggcctggtcaggacactgcccagtttggggagaatcaagctgatttttatcctgggacattgccaatttttcagctgcagcaattggacaaccagaaagactcctgtgggtgttgcggttgctgttcacatgaccccttcctgtgcatcccggcgtgggacacttgagcacattttcatgcatggcaagaatttccaggggaacccgcactttgtgggggcaccccgaaaggctgcggtggtgcgggtagagccctgtcacgtgtcccgtgccatcacatccagggatcgggcacttggtctccctcttttcaggccttggtgaatgtttattgttaaagatttgtcttccacccatgtcgataactttggtttgcctcctttcccctgctaggtgctccagcaggaacctatccagctctttgtaggtgttatggaaaacacaacctcgctcagcctgcagagcaattgcctgctccagcaaacttaaattccccttggccttttccaggtcactaccctcttccgtcattactgccaggctctcgctatcttcctcctcaacgtcagggaatgagggctgggcattgccatccaggggttctgcgagagcattctgcgggtctttcctttctgtttcagaatcacacctgttctcacaagggataaatttgtcaccttcagtttttatttcaggaacttccaataggtcttttttatgatctgttaaaacatactttgggactctaggtggtttggtttcttctgagaagttggagccactgtcccagccattttctgcactttcagagttactttcattgtcatcagaggagcagaagggtggctgagaatcatcaatcttgtctcttccatcatcagaatgaatcagaaagcactcgtctgcttcatcgctctctgcttttaaagactggatgccactgtcatttaaattttcacttacagtctgaacagatacatttttttcaaatttccccaagtgcattaaagacttgaccatgagctcttgataacaagagtatctgtcttccttcctactggagttttcttgtgcagttgaaagaagactttcatccataggttttatcatgatttcctctgcggtagagtgaccatgtgtttccaaggggccatcgtcctctgtcctgtcactgcggtcttcttggcagtctgcttttgggctgtagtgtcggggcttcattagcagggatttccttttgttgactggaacccccaaagcctgatcttcagctgttctcttctttgccatggagcaatcataggcaacactgagctcctggattagtgaatccattggcacctcggttcctttagagcgagtacgcagcgttttatcttcagcctctgcatccatcttccctaaaagctactggatctgaactggagagtttccatcactccttagtcttgatatgagcacgcagacacataaaatggaattgtcacaatgcttcagggacactcacaaaattgggggctcggtgcctcctagcctttgttctgcctctcacgctgacatcagggaagcagtgatgtagaataaagcaggggtgggctaggttagtccagtgtttgtgtcgttgtgtggtgtgcagggacactctgtgat

SEQ ID NO: 18697 - RNA, 4684 nt, Homo sapiens
  source 1..4684: mol_type = other RNA
tgagtgtgtgtgtgtgagtgtgtgtgtatattttgtagcatttgaagttttgtggcaagatttctatcaaattgaatgttgtcttgtttcctatggtgggtgagacccaaggtgccagtgtttgaagtaatcattcagattggagtagcattttttcatgtgttactatattttccattcctttccagtcaacccagtaagataaatgctatttcaggggatatggtatctacaaaatttttcatttggatgtgtttgtatttgctaagtacaaatctacaccaatattgtcacttgtatattgtaccaacatatggcaggaaagcctggctggtcacaccaagtcttatttttcatcttgggatacgagttgccaacgatctgatatgacttgaaaaacaaacagacaaatctgcatcactaaaaaggcttatgtttctttaaaacatttcaaataaataattcatattaacgaaaaccgtccagccaagtcgaatactttgctgattgctatatttaattattgctaacaaattctgagcaggctgttttccagcatcctgtgcttttgtgagtgcggattccccactagtgggcgccatttgtcttcttattccttccgtgcagctcaccttaccgcaaattcatttataaatacaaaaatcagtgaaaggtgggggaagaagtgtgcaataaaaatcaaactcaactatagtgcagtccttagacaaggatttccttcaccctttcctgtttcctcattaaaacccagcaagaaagatgacttgagaatagcatttctatttaaatcctattggaaaataaattaataaacacacttgtaaaaatacggcagacttcaaaatgcagttaaaagataaaaaactctttgattagtaataaataaattataaaaatgtcacatttattttacatatactttacaaaaaaaaaaagagtacaatgaagaaataaaagaaaaacatatgaaaataaataagatctaataattgactgcattgcttttaatccaagaagtctatcatagtttttctttcctttttatatcagctggggaaaataaaattagtgcaatgttgcaaattgtaaatgcagtacggcaacctccacgccttagcagtacatgaacctctaacagatccatctggagtttactgctgttggtaacttctgttgcccggcagcgctgtgatcctacacatggatacccttcactgcctgtttgatactttccagtagagctttgcattccggggaatagtcccgttccagattgctgtacatatctgtgagtgtatttacatatgcttcaaaattctgctcactgataggtcccatctgtggaagctggatgtcagcaaggcttgaaatgagagcttggcttagacctgccagctctttcagcagactttcattgttctgttctatgagtttgttctcctcctctatcgtctttaagttgctctccatagatgtgatctgggtctgaagtttcatcatatctgcttcaattttaaggttggattcattcagttcctttatttcttcatccaaatgcctaatttcttcatcactctctattcccccagttgctttgagcttgatggtcatgagttcttcagaaaccttgccctttttgataacttgtgcattgagaggacatccagataagcttcggtgggtgacaaaaacattatttacatggcccagcccattgcagcctggcaagggacaatgtggtagctcttgtttgttcagtttccaggagagggaggctccattgagaggattctccttctgtctcttggcagccagaggacagccagaagctgtgcggtgtgatgtgtatttacctgatatgtgaccttggccatcacaccctatcacaggacatttcagttcagggtcttctttttcttccttggtaggggtcattttgacaccacctttccttgcacgagggcatccggacaagcttctgtgggaagcatagtttccagtcacgtgccccgagccatcgcagcctggggttggacacttaagctcctgagagttggcagccatgagggattttagagtcttatctgctaaaggacatccagaaacactgcgatgagatgcatagtttcctgtcacgtggccacttccatcacatcctggtgttggacaggtgattagttcctttttgagatctcttgcatgaagcttgggtttagggcttggtatagaggcctctccaggaaactttttttcctctaaattttctagagagctcactgggtctttctctttctcctcctctgtcttcccgtgagttttgctatagttgataggagtgtcccagccctcttggtcacaaagagcctgatagaatgctgcattgaccagaatgctgcttgttttgaatggggaagaggaaggagttggaatagaagtgttagaggaagttaggggtgcagacttgtccaggattcgattttttttcatgcttaagtccaatgtgccattttcatccacttctatttcggctcccttggcatgcagactctgtggcttgttggagaggatgtctgtggcttccctgcagcgggtggaaaggttcaggatggcagcagctgctgctatgtgggtgtcttcactacattgaccgtagctataagagctggcacggccagggctctgggtgtgggcgcctgcactaggcagtcgattaggaaatttcactggatttggaaaatgctttgattcaggaaatggtggtgtttttcgtccttgcactgtttgtatgagagggcgtttaccgaaaacttgggcatcaaaactggcataatcaaatggtacttttccaaacttctcttgttcttttgacactgtggctctgggagaggtgatggcttgtgacgggaaattgaattcaatttgcttcaccaaacttgtcctgtgggcctggtcaggacactgcccagtttggggagaatcaagctgatttttatcctgggacattgccaatttttcagctgcagcaattggacaaccagaaagactcctgtgggtgttgcggttgctgttcacatgaccccttcctgtgcatcccggcgtgggacacttgagcacattttcatgcatggcaagaatttccaggggaacccgcactttgtgggggcaccccgaaaggctgcggtggtgcgggtagagccctgtcacgtgtcccgtgccatcacatccagggatcgggcacttggtctccctcttttcaggccttggtgaatgtttattgttaaagatttgtcttccacccatgtcgataactttggtttgcctcctttcccctgctaggtgctccagcaggaacctatccagctctttgtaggtgttatggaaaacacaacctcgctcagcctgcagagcaattgcctgctccagcaaacttaaattccccttggccttttccaggtcactaccctcttccgtcattactgccaggctctcgctatcttcctcctcaacgtcagggaatgagggctgggcattgccatccaggggttctgcgagagcattctgcgggtctttcctttctgtttcagaatcacacctgttctcacaagggataaatttgtcaccttcagtttttatttcaggaacttccaataggtcttttttatgatctgttaaaacatactttgggactctaggtggtttggtttcttctgagaagttggagccactgtcccagccattttctgcactttcagagttactttcattgtcatcagaggagcagaagggtggctgagaatcatcaatcttgtctcttccatcatcagaatgaatcagaaagcactcgtctgcttcatcgctctctgcttttaaagactggatgccactgtcatttaaattttcacttacagtctgaacagatacatttttttcaaatttccccaagtgcattaaagacttgaccatgagctcttgataacaagagtatctgtcttccttcctactggagttttcttgtgcagttgaaagaagactttcatccataggttttatcatgatttcctctgcggtagagtgaccatgtgtttccaaggggccatcgtcctctgtcctgtcactgcggtcttcttggcagtctgcttttgggctgtagtgtcggggcttcattagcagggatttccttttgttgactggaacccccaaagcctgatcttcagctgttctcttctttgccatggagcaatcataggcaacactgagctcctggattagtgaatccattggcacctcggttcctttagagcgagtacgcagcgttttatcttcagcctctgcatccatcttccctaaaagctactggatctgaactggagagtttccatcactccttagtcttgatatgagcacgcagacacataaaatggaattgtcacaatgcttcagggacactcacaaaattgggggctctttacctggcgaacgtctacaggtgtgtcgaaagttatcttttcctggatgtgttccaaaatgctcttatgctatttctcttaggatttctccacgctgccccattcagaaattttattattttctctagtattcccctgaggtcacattcagttaaaaacatcctgcccttctccctacaaaaaggttccatagaatc

SEQ ID NO: 18698 - RNA, 4583 nt, Homo sapiens
  source 1..4583: mol_type = other RNA
tgagtgtgtgtgtgtgagtgtgtgtgtatattttgtagcatttgaagttttgtggcaagatttctatcaaattgaatgttgtcttgtttcctatggtgggtgagacccaaggtgccagtgtttgaagtaatcattcagattggagtagcattttttcatgtgttactatattttccattcctttccagtcaacccagtaagataaatgctatttcaggggatatggtatctacaaaatttttcatttggatgtgtttgtatttgctaagtacaaatctacaccaatattgtcacttgtatattgtaccaacatatggcaggaaagcctggctggtcacaccaagtcttatttttcatcttgggatacgagttgccaacgatctgatatgacttgaaaaacaaacagacaaatctgcatcactaaaaaggcttatgtttctttaaaacatttcaaataaataattcatattaacgaaaaccgtccagccaagtcgaatactttgctgattgctatatttaattattgctaacaaattctgagcaggctgttttccagcatcctgtgcttttgtgagtgcggattccccactagtgggcgccatttgtcttcttattccttccgtgcagctcaccttaccgcaaattcatttataaatacaaaaatcagtgaaaggtgggggaagaagtgtgcaataaaaatcaaactcaactatagtgcagtccttagacaaggatttccttcaccctttcctgtttcctcattaaaacccagcaagaaagatgacttgagaatagcatttctatttaaatcctattggaaaataaattaataaacacacttgtaaaaatacggcagacttcaaaatgcagttaaaagataaaaaactctttgattagtaataaataaattataaaaatgtcacatttattttacatatactttacaaaaaaaaaaagagtacaatgaagaaataaaagaaaaacatatgaaaataaataagatctaataattgactgcattgcttttaatccaagaagtctatcatagtttttctttcctttttatatcagctggggaaaataaaattagtgcaatgttgcaaattgtaaatgcagtacggcaacctccacgccttagcagtacatgaacctctaacagatccatctggagtttactgctgttggtaacttctgttgcccggcagcgctgtgatcctacacatggatacccttcactgcctgtttgatactttccagtagagctttgcattccggggaatagtcccgttccagattgctgtacatatctgtgagtgtatttacatatgcttcaaaattctgctcactgataggtcccatctgtggaagctggatgtcagcaaggcttgaaatgagagcttggcttagacctgccagctctttcagcagactttcattgttctgttctatgagtttgttctcctcctctatcgtctttaagttgctctccatagatgtgatctgggtctgaagtttcatcatatctgcttcaattttaaggttggattcattcagttcctttatttcttcatccaaatgcctaatttcttcatcactctctattcccccagttgctttgagcttgatggtcatgagttcttcagaaaccttgccctttttgataacttgtgcattgagaggacatccagataagcttcggtgggtgacaaaaacattatttacatggcccagcccattgcagcctggcaagggacaatgtggtagctcttgtttgttcagtttccaggagagggaggctccattgagaggattctccttctgtctcttggcagccagaggacagccagaagctgtgcggtgtgatgtgtatttacctgatatgtgaccttggccatcacaccctatcacaggacatttcagttcagggtcttctttttcttccttggtaggggtcattttgacaccacctttccttgcacgagggcatccggacaagcttctgtgggaagcatagtttccagtcacgtgccccgagccatcgcagcctggggttggacacttaagctcctgagagttggcagccatgagggattttagagtcttatctgctaaaggacatccagaaacactgcgatgagatgcatagtttcctgtcacgtggccacttccatcacatcctggtgttggacaggtgattagttcctttttgagatctcttgcatgaagcttgggtttagggcttggtatagaggcctctccaggaaactttttttcctctaaattttctagagagctcactgggtctttctctttctcctcctctgtcttcccgtgagttttgctatagttgataggagtgtcccagccctcttggtcacaaagagcctgatagaatgctgcattgaccagaatgctgcttgttttgaatggggaagaggaaggagttggaatagaagtgttagaggaagttaggggtgcagacttgtccaggattcgattttttttcatgcttaagtccaatgtgccattttcatccacttctatttcggctcccttggcatgcagactctgtggcttgttggagaggatgtctgtggcttccctgcagcgggtggaaaggttcaggatggcagcagctgctgctatgtgggtgtcttcactacattgaccgtagctataagagctggcacggccagggctctgggtgtgggcgcctgcactaggcagtcgattaggaaatttcactggatttggaaaatgctttgattcaggaaatggtggtgtttttcgtccttgcactgtttgtatgagagggcgtttaccgaaaacttgggcatcaaaactggcataatcaaatggtacttttccaaacttctcttgttcttttgacactgtggctctgggagaggtgatggcttgtgacgggaaattgaattcaatttgcttcaccaaacttgtcctgtgggcctggtcaggacactgcccagtttggggagaatcaagctgatttttatcctgggacattgccaatttttcagctgcagcaattggacaaccagaaagactcctgtgggtgttgcggttgctgttcacatgaccccttcctgtgcatcccggcgtgggacacttgagcacattttcatgcatggcaagaatttccaggggaacccgcactttgtgggggcaccccgaaaggctgcggtggtgcgggtagagccctgtcacgtgtcccgtgccatcacatccagggatcgggcacttggtctccctcttttcaggccttggtgaatgtttattgttaaagatttgtcttccacccatgtcgataactttggtttgcctcctttcccctgctaggtgctccagcaggaacctatccagctctttgtaggtgttatggaaaacacaacctcgctcagcctgcagagcaattgcctgctccagcaaacttaaattccccttggccttttccaggtcactaccctcttccgtcattactgccaggctctcgctatcttcctcctcaacgtcagggaatgagggctgggcattgccatccaggggttctgcgagagcattctgcgggtctttcctttctgtttcagaatcacacctgttctcacaagggataaatttgtcaccttcagtttttatttcaggaacttccaataggtcttttttatgatctgttaaaacatactttgggactctaggtggtttggtttcttctgagaagttggagccactgtcccagccattttctgcactttcagagttactttcattgtcatcagaggagcagaagggtggctgagaatcatcaatcttgtctcttccatcatcagaatgaatcagaaagcactcgtctgcttcatcgctctctgcttttaaagactggatgccactgtcatttaaattttcacttacagtctgaacagatacatttttttcaaatttccccaagtgcattaaagacttgaccatgagctcttgataacaagagtatctgtcttccttcctactggagttttcttgtgcagttgaaagaagactttcatccataggttttatcatgatttcctctgcggtagagtgaccatgtgtttccaaggggccatcgtcctctgtcctgtcactgcggtcttcttggcagtctgcttttgggctgtagtgtcggggcttcattagcagggatttccttttgttgactggaacccccaaagcctgatcttcagctgttctcttctttgccatggagcaatcataggcaacactgagctcctggattagtgaatccattggcacctcggttcctttagagcgagtacgcagcgttttatcttcagcctctgcatccatcttccctaaaagctactggatctgaactggagagtttccatcactccttagtcttgatatgagcacgcagacacataaaatggaattgtcacaatgcttcagggacactcacaaaattgggggctttttttgtttgtttccaaaacttatatttctctcctccctggtgggctgaacggaaacactaaagctgtttctttgaaaggtagttcccatgatatgac

SEQ ID NO: 18699 - RNA, 4605 nt, Homo sapiens
  source 1..4605: mol_type = other RNA
tgagtgtgtgtgtgtgagtgtgtgtgtatattttgtagcatttgaagttttgtggcaagatttctatcaaattgaatgttgtcttgtttcctatggtgggtgagacccaaggtgccagtgtttgaagtaatcattcagattggagtagcattttttcatgtgttactatattttccattcctttccagtcaacccagtaagataaatgctatttcaggggatatggtatctacaaaatttttcatttggatgtgtttgtatttgctaagtacaaatctacaccaatattgtcacttgtatattgtaccaacatatggcaggaaagcctggctggtcacaccaagtcttatttttcatcttgggatacgagttgccaacgatctgatatgacttgaaaaacaaacagacaaatctgcatcactaaaaaggcttatgtttctttaaaacatttcaaataaataattcatattaacgaaaaccgtccagccaagtcgaatactttgctgattgctatatttaattattgctaacaaattctgagcaggctgttttccagcatcctgtgcttttgtgagtgcggattccccactagtgggcgccatttgtcttcttattccttccgtgcagctcaccttaccgcaaattcatttataaatacaaaaatcagtgaaaggtgggggaagaagtgtgcaataaaaatcaaactcaactatagtgcagtccttagacaaggatttccttcaccctttcctgtttcctcattaaaacccagcaagaaagatgacttgagaatagcatttctatttaaatcctattggaaaataaattaataaacacacttgtaaaaatacggcagacttcaaaatgcagttaaaagataaaaaactctttgattagtaataaataaattataaaaatgtcacatttattttacatatactttacaaaaaaaaaaagagtacaatgaagaaataaaagaaaaacatatgaaaataaataagatctaataattgactgcattgcttttaatccaagaagtctatcatagtttttctttcctttttatatcagctggggaaaataaaattagtgcaatgttgcaaattgtaaatgcagtacggcaacctccacgccttagcagtacatgaacctctaacagatccatctggagtttactgctgttggtaacttctgttgcccggcagcgctgtgatcctacacatggatacccttcactgcctgtttgatactttccagtagagctttgcattccggggaatagtcccgttccagattgctgtacatatctgtgagtgtatttacatatgcttcaaaattctgctcactgataggtcccatctgtggaagctggatgtcagcaaggcttgaaatgagagcttggcttagacctgccagctctttcagcagactttcattgttctgttctatgagtttgttctcctcctctatcgtctttaagttgctctccatagatgtgatctgggtctgaagtttcatcatatctgcttcaattttaaggttggattcattcagttcctttatttcttcatccaaatgcctaatttcttcatcactctctattcccccagttgctttgagcttgatggtcatgagttcttcagaaaccttgccctttttgataacttgtgcattgagaggacatccagataagcttcggtgggtgacaaaaacattatttacatggcccagcccattgcagcctggcaagggacaatgtggtagctcttgtttgttcagtttccaggagagggaggctccattgagaggattctccttctgtctcttggcagccagaggacagccagaagctgtgcggtgtgatgtgtatttacctgatatgtgaccttggccatcacaccctatcacaggacatttcagttcagggtcttctttttcttccttggtaggggtcattttgacaccacctttccttgcacgagggcatccggacaagcttctgtgggaagcatagtttccagtcacgtgccccgagccatcgcagcctggggttggacacttaagctcctgagagttggcagccatgagggattttagagtcttatctgctaaaggacatccagaaacactgcgatgagatgcatagtttcctgtcacgtggccacttccatcacatcctggtgttggacaggtgattagttcctttttgagatctcttgcatgaagcttgggtttagggcttggtatagaggcctctccaggaaactttttttcctctaaattttctagagagctcactgggtctttctctttctcctcctctgtcttcccgtgagttttgctatagttgataggagtgtcccagccctcttggtcacaaagagcctgatagaatgctgcattgaccagaatgctgcttgttttgaatggggaagaggaaggagttggaatagaagtgttagaggaagttaggggtgcagacttgtccaggattcgattttttttcatgcttaagtccaatgtgccattttcatccacttctatttcggctcccttggcatgcagactctgtggcttgttggagaggatgtctgtggcttccctgcagcgggtggaaaggttcaggatggcagcagctgctgctatgtgggtgtcttcactacattgaccgtagctataagagctggcacggccagggctctgggtgtgggcgcctgcactaggcagtcgattaggaaatttcactggatttggaaaatgctttgattcaggaaatggtggtgtttttcgtccttgcactgtttgtatgagagggcgtttaccgaaaacttgggcatcaaaactggcataatcaaatggtacttttccaaacttctcttgttcttttgacactgtggctctgggagaggtgatggcttgtgacgggaaattgaattcaatttgcttcaccaaacttgtcctgtgggcctggtcaggacactgcccagtttggggagaatcaagctgatttttatcctgggacattgccaatttttcagctgcagcaattggacaaccagaaagactcctgtgggtgttgcggttgctgttcacatgaccccttcctgtgcatcccggcgtgggacacttgagcacattttcatgcatggcaagaatttccaggggaacccgcactttgtgggggcaccccgaaaggctgcggtggtgcgggtagagccctgtcacgtgtcccgtgccatcacatccagggatcgggcacttggtctccctcttttcaggccttggtgaatgtttattgttaaagatttgtcttccacccatgtcgataactttggtttgcctcctttcccctgctaggtgctccagcaggaacctatccagctctttgtaggtgttatggaaaacacaacctcgctcagcctgcagagcaattgcctgctccagcaaacttaaattccccttggccttttccaggtcactaccctcttccgtcattactgccaggctctcgctatcttcctcctcaacgtcagggaatgagggctgggcattgccatccaggggttctgcgagagcattctgcgggtctttcctttctgtttcagaatcacacctgttctcacaagggataaatttgtcaccttcagtttttatttcaggaacttccaataggtcttttttatgatctgttaaaacatactttgggactctaggtggtttggtttcttctgagaagttggagccactgtcccagccattttctgcactttcagagttactttcattgtcatcagaggagcagaagggtggctgagaatcatcaatcttgtctcttccatcatcagaatgaatcagaaagcactcgtctgcttcatcgctctctgcttttaaagactggatgccactgtcatttaaattttcacttacagtctgaacagatacatttttttcaaatttccccaagtgcattaaagacttgaccatgagctcttgataacaagagtatctgtcttccttcctactggagttttcttgtgcagttgaaagaagactttcatccataggttttatcatgatttcctctgcggtagagtgaccatgtgtttccaaggggccatcgtcctctgtcctgtcactgcggtcttcttggcagtctgcttttgggctgtagtgtcggggcttcattagcagggatttccttttgttgactggaacccccaaagcctgatcttcagctgttctcttctttgccatggagcaatcataggcaacactgagctcctggattagtgaatccattggcacctcggttcctttagagcgagtacgcagcgttttatcttcagcctctgcatccatcttccctaaaagctactggatctgaactggagagtttccatcactcctttacctggcgaacgtctacaggtgtgtcgaaagttatcttttcctggatgtgttccaaaatgctcttatgctatttctcttaggatttctccacgctgccccattcagaaattttattattttctctagtattcccctgaggtcacattcagttaaaaacatcctgcccttctccctacaaaaaggttccatagaatc

SEQ ID NO: 18700 - RNA, 4504 nt, Homo sapiens
  source 1..4504: mol_type = other RNA
tgagtgtgtgtgtgtgagtgtgtgtgtatattttgtagcatttgaagttttgtggcaagatttctatcaaattgaatgttgtcttgtttcctatggtgggtgagacccaaggtgccagtgtttgaagtaatcattcagattggagtagcattttttcatgtgttactatattttccattcctttccagtcaacccagtaagataaatgctatttcaggggatatggtatctacaaaatttttcatttggatgtgtttgtatttgctaagtacaaatctacaccaatattgtcacttgtatattgtaccaacatatggcaggaaagcctggctggtcacaccaagtcttatttttcatcttgggatacgagttgccaacgatctgatatgacttgaaaaacaaacagacaaatctgcatcactaaaaaggcttatgtttctttaaaacatttcaaataaataattcatattaacgaaaaccgtccagccaagtcgaatactttgctgattgctatatttaattattgctaacaaattctgagcaggctgttttccagcatcctgtgcttttgtgagtgcggattccccactagtgggcgccatttgtcttcttattccttccgtgcagctcaccttaccgcaaattcatttataaatacaaaaatcagtgaaaggtgggggaagaagtgtgcaataaaaatcaaactcaactatagtgcagtccttagacaaggatttccttcaccctttcctgtttcctcattaaaacccagcaagaaagatgacttgagaatagcatttctatttaaatcctattggaaaataaattaataaacacacttgtaaaaatacggcagacttcaaaatgcagttaaaagataaaaaactctttgattagtaataaataaattataaaaatgtcacatttattttacatatactttacaaaaaaaaaaagagtacaatgaagaaataaaagaaaaacatatgaaaataaataagatctaataattgactgcattgcttttaatccaagaagtctatcatagtttttctttcctttttatatcagctggggaaaataaaattagtgcaatgttgcaaattgtaaatgcagtacggcaacctccacgccttagcagtacatgaacctctaacagatccatctggagtttactgctgttggtaacttctgttgcccggcagcgctgtgatcctacacatggatacccttcactgcctgtttgatactttccagtagagctttgcattccggggaatagtcccgttccagattgctgtacatatctgtgagtgtatttacatatgcttcaaaattctgctcactgataggtcccatctgtggaagctggatgtcagcaaggcttgaaatgagagcttggcttagacctgccagctctttcagcagactttcattgttctgttctatgagtttgttctcctcctctatcgtctttaagttgctctccatagatgtgatctgggtctgaagtttcatcatatctgcttcaattttaaggttggattcattcagttcctttatttcttcatccaaatgcctaatttcttcatcactctctattcccccagttgctttgagcttgatggtcatgagttcttcagaaaccttgccctttttgataacttgtgcattgagaggacatccagataagcttcggtgggtgacaaaaacattatttacatggcccagcccattgcagcctggcaagggacaatgtggtagctcttgtttgttcagtttccaggagagggaggctccattgagaggattctccttctgtctcttggcagccagaggacagccagaagctgtgcggtgtgatgtgtatttacctgatatgtgaccttggccatcacaccctatcacaggacatttcagttcagggtcttctttttcttccttggtaggggtcattttgacaccacctttccttgcacgagggcatccggacaagcttctgtgggaagcatagtttccagtcacgtgccccgagccatcgcagcctggggttggacacttaagctcctgagagttggcagccatgagggattttagagtcttatctgctaaaggacatccagaaacactgcgatgagatgcatagtttcctgtcacgtggccacttccatcacatcctggtgttggacaggtgattagttcctttttgagatctcttgcatgaagcttgggtttagggcttggtatagaggcctctccaggaaactttttttcctctaaattttctagagagctcactgggtctttctctttctcctcctctgtcttcccgtgagttttgctatagttgataggagtgtcccagccctcttggtcacaaagagcctgatagaatgctgcattgaccagaatgctgcttgttttgaatggggaagaggaaggagttggaatagaagtgttagaggaagttaggggtgcagacttgtccaggattcgattttttttcatgcttaagtccaatgtgccattttcatccacttctatttcggctcccttggcatgcagactctgtggcttgttggagaggatgtctgtggcttccctgcagcgggtggaaaggttcaggatggcagcagctgctgctatgtgggtgtcttcactacattgaccgtagctataagagctggcacggccagggctctgggtgtgggcgcctgcactaggcagtcgattaggaaatttcactggatttggaaaatgctttgattcaggaaatggtggtgtttttcgtccttgcactgtttgtatgagagggcgtttaccgaaaacttgggcatcaaaactggcataatcaaatggtacttttccaaacttctcttgttcttttgacactgtggctctgggagaggtgatggcttgtgacgggaaattgaattcaatttgcttcaccaaacttgtcctgtgggcctggtcaggacactgcccagtttggggagaatcaagctgatttttatcctgggacattgccaatttttcagctgcagcaattggacaaccagaaagactcctgtgggtgttgcggttgctgttcacatgaccccttcctgtgcatcccggcgtgggacacttgagcacattttcatgcatggcaagaatttccaggggaacccgcactttgtgggggcaccccgaaaggctgcggtggtgcgggtagagccctgtcacgtgtcccgtgccatcacatccagggatcgggcacttggtctccctcttttcaggccttggtgaatgtttattgttaaagatttgtcttccacccatgtcgataactttggtttgcctcctttcccctgctaggtgctccagcaggaacctatccagctctttgtaggtgttatggaaaacacaacctcgctcagcctgcagagcaattgcctgctccagcaaacttaaattccccttggccttttccaggtcactaccctcttccgtcattactgccaggctctcgctatcttcctcctcaacgtcagggaatgagggctgggcattgccatccaggggttctgcgagagcattctgcgggtctttcctttctgtttcagaatcacacctgttctcacaagggataaatttgtcaccttcagtttttatttcaggaacttccaataggtcttttttatgatctgttaaaacatactttgggactctaggtggtttggtttcttctgagaagttggagccactgtcccagccattttctgcactttcagagttactttcattgtcatcagaggagcagaagggtggctgagaatcatcaatcttgtctcttccatcatcagaatgaatcagaaagcactcgtctgcttcatcgctctctgcttttaaagactggatgccactgtcatttaaattttcacttacagtctgaacagatacatttttttcaaatttccccaagtgcattaaagacttgaccatgagctcttgataacaagagtatctgtcttccttcctactggagttttcttgtgcagttgaaagaagactttcatccataggttttatcatgatttcctctgcggtagagtgaccatgtgtttccaaggggccatcgtcctctgtcctgtcactgcggtcttcttggcagtctgcttttgggctgtagtgtcggggcttcattagcagggatttccttttgttgactggaacccccaaagcctgatcttcagctgttctcttctttgccatggagcaatcataggcaacactgagctcctggattagtgaatccattggcacctcggttcctttagagcgagtacgcagcgttttatcttcagcctctgcatccatcttccctaaaagctactggatctgaactggagagtttccatcactcttttttgtttgtttccaaaacttatatttctctcctccctggtgggctgaacggaaacactaaagctgtttctttgaaaggtagttcccatgatatgac

SEQ ID NO: 18701 - RNA, 5161 nt, Homo sapiens
  source 1..5161: mol_type = other RNA
tgagtgtgtgtgtgtgagtgtgtgtgtatattttgtagcatttgaagttttgtggcaagatttctatcaaattgaatgttgtcttgtttcctatggtgggtgagacccaaggtgccagtgtttgaagtaatcattcagattggagtagcattttttcatgtgttactatattttccattcctttccagtcaacccagtaagataaatgctatttcaggggatatggtatctacaaaatttttcatttggatgtgtttgtatttgctaagtacaaatctacaccaatattgtcacttgtatattgtaccaacatatggcaggaaagcctggctggtcacaccaagtcttatttttcatcttgggatacgagttgccaacgatctgatatgacttgaaaaacaaacagacaaatctgcatcactaaaaaggcttatgtttctttaaaacatttcaaataaataattcatattaacgaaaaccgtccagccaagtcgaatactttgctgattgctatatttaattattgctaacaaattctgagcaggctgttttccagcatcctgtgcttttgtgagtgcggattccccactagtgggcgccatttgtcttcttattccttccgtgcagctcaccttaccgcaaattcatttataaatacaaaaatcagtgaaaggtgggggaagaagtgtgcaataaaaatcaaactcaactatagtgcagtccttagacaaggatttccttcaccctttcctgtttcctcattaaaacccagcaagaaagatgacttgagaatagcatttctatttaaatcctattggaaaataaattaataaacacacttgtaaaaatacggcagacttcaaaatgcagttaaaagataaaaaactctttgattagtaataaataaattataaaaatgtcacatttattttacatatactttacaaaaaaaaaaagagtacaatgaagaaataaaagaaaaacatatgaaaataaataagatctaataattgactgcattgcttttaatccaagaagtctatcatagtttttctttcctttttatatcagctggggaaaataaaattagtgcaatgttgcaaattgtaaatgcagtacggcaacctccacgccttagcagtacatgaacctctaacagatccatctggagtttactgctgttggtaacttctgttgcccggcagcgctgtgatcctacacatggatacccttcactgcctgtttgatactttccagtagagctttgcattccggggaatagtcccgttccagattgctgtacatatctgtgagtgtatttacatatgcttcaaaattctgctcactgataggtcccatctgtggaagctggatgtcagcaaggcttgaaatgagagcttggcttagacctgccagctctttcagcagactttcattgttctgttctatgagtttgttctcctcctctatcgtctttaagttgctctccatagatgtgatctgggtctgaagtttcatcatatctgcttcaattttaaggttggattcattcagttcctttatttcttcatccaaatgcctaatttcttcatcactctctattcccccagttgctttgagcttgatggtcatgagttcttcagaaaccttgccctttttgataacttgtgcattgagaggacatccagataagcttcggtgggtgacaaaaacattatttacatggcccagcccattgcagcctggcaagggacaatgtggtagctcttgtttgttcagtttccaggagagggaggctccattgagaggattctccttctgtctcttggcagccagaggacagccagaagctgtgcggtgtgatgtgtatttacctgatatgtgaccttggccatcacaccctatcacaggacatttcagttcagggtcttctttttcttccttggtaggggtcattttgacaccacctttccttgcacgagggcatccggacaagcttctgtgggaagcatagtttccagtcacgtgccccgagccatcgcagcctggggttggacacttaagctcctgagagttggcagccatgagggattttagagtcttatctgctaaaggacatccagaaacactgcgatgagatgcatagtttcctgtcacgtggccacttccatcacatcctggtgttggacaggtgattagttcctttttgagatctcttgcatgaagcttgggtttagggcttggtatagaggcctctccaggaaactttttttcctctaaattttctagagagctcactgggtctttctctttctcctcctctgtcttcccgtgagttttgctatagttgataggagtgtcccagccctcttggtcacaaagagcctgatagaatgctgcattgaccagaatgctgcttgttttgaatggggaagaggaaggagttggaatagaagtgttagaggaagttaggggtgcagacttgtccaggattcgattttttttcatgcttaagtccaatgtgccattttcatccacttctatttcggctcccttggcatgcagactctgtggcttgttggagaggatgtctgtggcttccctgcagcgggtggaaaggttcaggatggcagcagctgctgctatgtgggtgtcttcactacattgaccgtagctataagagctggcacggccagggctctgggtgtgggcgcctgcactaggcagtcgattaggaaatttcactggatttggaaaatgctttgattcaggaaatggtggtgtttttcgtccttgcactgtttgtatgagagggcgtttaccgaaaacttgggcatcaaaactggcataatcaaatggtacttttccaaacttctcttgttcttttgacactgtggctctgggagaggtgatggcttgtgacgggaaattgaattcaatttgcttcaccaaacttgtcctgtgggcctggtcaggacactgcccagtttggggagaatcaagctgatttttatcctgggacattgccaatttttcagctgcagcaattggacaaccagaaagactcctgtgggtgttgcggttgctgttcacatgaccccttcctgtgcatcccggcgtgggacacttgagcacattttcatgcatggcaagaatttccaggggaacccgcactttgtgggggcaccccgaaaggctgcggtggtgcgggtagagccctgtcacgtgtcccgtgccatcacatccagggatcgggcacttggtctccctcttttcaggccttggtgaatgtttattgttaaagatttgtcttccacccatgtcgataactttggtttgcctcctttcccctgctaggtgctccagcaggaacctatccagctctttgtaggtgttatggaaaacacaacctcgctcagcctgcagagcaattgcctgctccagcaaacttaaattccccttggccttttccaggtcactaccctcttccgtcattactgccaggctctcgctatcttcctcctcaacgtcagggaatgagggctgggcattgccatccaggggttctgcgagagcattctgcgggtctttcctttctgtttcagaatcacacctgttctcacaagggataaatttgtcaccttcagtttttatttcaggaacttccaataggtcttttttatgatctgttaaaacatactttgggactctaggtggtttggtttcttctgagaagttggagccactgtcccagccattttctgcactttcagagttactttcattgtcatcagaggagcagaagggtggctgagaatcatcaatcttgtctcttccatcatcagaatgaatcagaaagcactcgtctgcttcatcgctctctgcttttaaagactggatgccactgtcatttaaattttcacttacagtctgaacagatacatttttttcaaatttccccaagtgcattaaagacttgaccatgagctcttgataacaagagtatctgtcttccttcctactggagttttcttgtgcagttgaaagaagactttcatccataggttttatcatgatttcctctgcggtagagtgaccatgtgtttccaaggggccatcgtcctctgtcctgtcactgcggtcttcttggcagtctgcttttgggctgtagtgtcggggcttcattagcagggatttccttttgttgactggaacccccaaagcctgatcttcagctgttctcttctttgccatggagcaatcataggcaacacttgagcactttgtgagtctaggagtctacttctctctattctcacaggggcaatctgagctcctggattagtgaatccattggcacctcggttcctttagagcgagtacgcagcgttttatcttcagcctctgcatccataaacctataaacagatgtataaagtgatttcctagtacttgtacttgacgtcttttcttactggagcttacatcaggggcaataagcaggtctcttccacatcgccccagtgcacagatctggtaccttcttttaggctgaagaggaagtcctggaattgctctctttttctccaggtaacttgtatgtcaactcagtttgccctgctgtgtcagggggactaaataaatgactttgtcttatttagtgataaatcctgaaattcattctttcttgcagaaaatttctaccgtcctgccttctctaccctttgcagtatatcaaagtgctcagctttttaatcatagatttctgtgtttcttgtaggatttgaccagacattaaatagatgcttcttcaacttaagtcagcaactgtagttccttccctaaaagctactggatctgaactggagagtttccatcactccttagtcttgatatgagcacgcagacacataaaatggaattgtcacaatgcttcagggacactcacaaaattgggggctctttacctggcgaacgtctacaggtgtgtcgaaagttatcttttcctggatgtgttccaaaatgctcttatgctatttctcttaggatttctccacgctgccccattcagaaattttattattttctctagtattcccctgaggtcacattcagttaaaaacatcctgcccttctccctacaaaaaggttccatagaatc

SEQ ID NO: 18702 - RNA, 5112 nt, Homo sapiens
  source 1..5112: mol_type = other RNA
tgagtgtgtgtgtgtgagtgtgtgtgtatattttgtagcatttgaagttttgtggcaagatttctatcaaattgaatgttgtcttgtttcctatggtgggtgagacccaaggtgccagtgtttgaagtaatcattcagattggagtagcattttttcatgtgttactatattttccattcctttccagtcaacccagtaagataaatgctatttcaggggatatggtatctacaaaatttttcatttggatgtgtttgtatttgctaagtacaaatctacaccaatattgtcacttgtatattgtaccaacatatggcaggaaagcctggctggtcacaccaagtcttatttttcatcttgggatacgagttgccaacgatctgatatgacttgaaaaacaaacagacaaatctgcatcactaaaaaggcttatgtttctttaaaacatttcaaataaataattcatattaacgaaaaccgtccagccaagtcgaatactttgctgattgctatatttaattattgctaacaaattctgagcaggctgttttccagcatcctgtgcttttgtgagtgcggattccccactagtgggcgccatttgtcttcttattccttccgtgcagctcaccttaccgcaaattcatttataaatacaaaaatcagtgaaaggtgggggaagaagtgtgcaataaaaatcaaactcaactatagtgcagtccttagacaaggatttccttcaccctttcctgtttcctcattaaaacccagcaagaaagatgacttgagaatagcatttctatttaaatcctattggaaaataaattaataaacacacttgtaaaaatacggcagacttcaaaatgcagttaaaagataaaaaactctttgattagtaataaataaattataaaaatgtcacatttattttacatatactttacaaaaaaaaaaagagtacaatgaagaaataaaagaaaaacatatgaaaataaataagatctaataattgactgcattgcttttaatccaagaagtctatcatagtttttctttcctttttatatcagctggggaaaataaaattagtgcaatgttgcaaattgtaaatgcagtacggcaacctccacgccttagcagtacatgaacctctaacagatccatctggagtttactgctgttggtaacttctgttgcccggcagcgctgtgatcctacacatggatacccttcactgcctgtttgatactttccagtagagctttgcattccggggaatagtcccgttccagattgctgtacatatctgtgagtgtatttacatatgcttcaaaattctgctcactgataggtcccatctgtggaagctggatgtcagcaaggcttgaaatgagagcttggcttagacctgccagctctttcagcagactttcattgttctgttctatgagtttgttctcctcctctatcgtctttaagttgctctccatagatgtgatctgggtctgaagtttcatcatatctgcttcaattttaaggttggattcattcagttcctttatttcttcatccaaatgcctaatttcttcatcactctctattcccccagttgctttgagcttgatggtcatgagttcttcagaaaccttgccctttttgataacttgtgcattgagaggacatccagataagcttcggtgggtgacaaaaacattatttacatggcccagcccattgcagcctggcaagggacaatgtggtagctcttgtttgttcagtttccaggagagggaggctccattgagaggattctccttctgtctcttggcagccagaggacagccagaagctgtgcggtgtgatgtgtatttacctgatatgtgaccttggccatcacaccctatcacaggacatttcagttcagggtcttctttttcttccttggtaggggtcattttgacaccacctttccttgcacgagggcatccggacaagcttctgtgggaagcatagtttccagtcacgtgccccgagccatcgcagcctggggttggacacttaagctcctgagagttggcagccatgagggattttagagtcttatctgctaaaggacatccagaaacactgcgatgagatgcatagtttcctgtcacgtggccacttccatcacatcctggtgttggacaggtgattagttcctttttgagatctcttgcatgaagcttgggtttagggcttggtatagaggcctctccaggaaactttttttcctctaaattttctagagagctcactgggtctttctctttctcctcctctgtcttcccgtgagttttgctatagttgataggagtgtcccagccctcttggtcacaaagagcctgatagaatgctgcattgaccagaatgctgcttgttttgaatggggaagaggaaggagttggaatagaagtgttagaggaagttaggggtgcagacttgtccaggattcgattttttttcatgcttaagtccaatgtgccattttcatccacttctatttcggctcccttggcatgcagactctgtggcttgttggagaggatgtctgtggcttccctgcagcgggtggaaaggttcaggatggcagcagctgctgctatgtgggtgtcttcactacattgaccgtagctataagagctggcacggccagggctctgggtgtgggcgcctgcactaggcagtcgattaggaaatttcactggatttggaaaatgctttgattcaggaaatggtggtgtttttcgtccttgcactgtttgtatgagagggcgtttaccgaaaacttgggcatcaaaactggcataatcaaatggtacttttccaaacttctcttgttcttttgacactgtggctctgggagaggtgatggcttgtgacgggaaattgaattcaatttgcttcaccaaacttgtcctgtgggcctggtcaggacactgcccagtttggggagaatcaagctgatttttatcctgggacattgccaatttttcagctgcagcaattggacaaccagaaagactcctgtgggtgttgcggttgctgttcacatgaccccttcctgtgcatcccggcgtgggacacttgagcacattttcatgcatggcaagaatttccaggggaacccgcactttgtgggggcaccccgaaaggctgcggtggtgcgggtagagccctgtcacgtgtcccgtgccatcacatccagggatcgggcacttggtctccctcttttcaggccttggtgaatgtttattgttaaagatttgtcttccacccatgtcgataactttggtttgcctcctttcccctgctaggtgctccagcaggaacctatccagctctttgtaggtgttatggaaaacacaacctcgctcagcctgcagagcaattgcctgctccagcaaacttaaattccccttggccttttccaggtcactaccctcttccgtcattactgccaggctctcgctatcttcctcctcaacgtcagggaatgagggctgggcattgccatccaggggttctgcgagagcattctgcgggtctttcctttctgtttcagaatcacacctgttctcacaagggataaatttgtcaccttcagtttttatttcaggaacttccaataggtcttttttatgatctgttaaaacatactttgggactctaggtggtttggtttcttctgagaagttggagccactgtcccagccattttctgcactttcagagttactttcattgtcatcagaggagcagaagggtggctgagaatcatcaatcttgtctcttccatcatcagaatgaatcagaaagcactcgtctgcttcatcgctctctgcttttaaagactggatgccactgtcatttaaattttcacttacagtctgaacagatacatttttttcaaatttccccaagtgcattaaagacttgaccatgagctcttgataacaagagtatctgtcttccttcctactggagttttcttgtgcagttgaaagaagactttcatccataggttttatcatgatttcctctgcggtagagtgaccatgtgtttccaaggggccatcgtcctctgtcctgtcactgcggtcttcttggcagtctgcttttgggctgtagtgtcggggcttcattagcagggatttccttttgttgactggaacccccaaagcctgatcttcagctgttctcttctttgccatggagcaatcataggcaacacttggggaatccagtgtcagagactggggtgttgagaaaccagcaaggagacctgagaagatgcagtctgagaggtagaggaaaccagggaggttgcaatgttgggaagccaagtttctttgacaatggccagggttgtgtgagccttccagcttttccttcaagaacgcagagcttgctgatcttccaggacagactgtaggctctgggtcagcttccaaagaccaggaggatggtccttaggggctcgagagaattaccttgagcactttgtgagtctaggagtctacttctctctattctcacaggggcaatctgagctcctggattagtgaatccattggcacctcggttcctttagagcgagtacgcagcgttttatcttcagcctctgcatccatctctctttttctccaggtaacttgtatgtcaactcagtttgccctgctgtgtcagggggactaaataaatgactttgtcttatttagtgataaatcctgaaattcattctttcttgcagaaaatttctaccgtcctgccttctctaccctttgcagtatatcaaagtgctcagctttttaatcatagatttctgtgtttcttgtaggatttgaccagacattaaatagatgcttcttcaacttaagtcagcaactgtagttccttccctaaaagctactggatctgaactggagagtttccatcactccggtgcctcctagcctttgttctgcctctcacgctgacatcagggaagcagtgatgtagaataaagcaggggtgggctaggttagtccagtgtttgtgtcgttgtgtggtgtgcagggacactctgtgat

SEQ ID NO: 18703 - RNA, 5093 nt, Homo sapiens
  source 1..5093: mol_type = other RNA
tgagtgtgtgtgtgtgagtgtgtgtgtatattttgtagcatttgaagttttgtggcaagatttctatcaaattgaatgttgtcttgtttcctatggtgggtgagacccaaggtgccagtgtttgaagtaatcattcagattggagtagcattttttcatgtgttactatattttccattcctttccagtcaacccagtaagataaatgctatttcaggggatatggtatctacaaaatttttcatttggatgtgtttgtatttgctaagtacaaatctacaccaatattgtcacttgtatattgtaccaacatatggcaggaaagcctggctggtcacaccaagtcttatttttcatcttgggatacgagttgccaacgatctgatatgacttgaaaaacaaacagacaaatctgcatcactaaaaaggcttatgtttctttaaaacatttcaaataaataattcatattaacgaaaaccgtccagccaagtcgaatactttgctgattgctatatttaattattgctaacaaattctgagcaggctgttttccagcatcctgtgcttttgtgagtgcggattccccactagtgggcgccatttgtcttcttattccttccgtgcagctcaccttaccgcaaattcatttataaatacaaaaatcagtgaaaggtgggggaagaagtgtgcaataaaaatcaaactcaactatagtgcagtccttagacaaggatttccttcaccctttcctgtttcctcattaaaacccagcaagaaagatgacttgagaatagcatttctatttaaatcctattggaaaataaattaataaacacacttgtaaaaatacggcagacttcaaaatgcagttaaaagataaaaaactctttgattagtaataaataaattataaaaatgtcacatttattttacatatactttacaaaaaaaaaaagagtacaatgaagaaataaaagaaaaacatatgaaaataaataagatctaataattgactgcattgcttttaatccaagaagtctatcatagtttttctttcctttttatatcagctggggaaaataaaattagtgcaatgttgcaaattgtaaatgcagtacggcaacctccacgccttagcagtacatgaacctctaacagatccatctggagtttactgctgttggtaacttctgttgcccggcagcgctgtgatcctacacatggatacccttcactgcctgtttgatactttccagtagagctttgcattccggggaatagtcccgttccagattgctgtacatatctgtgagtgtatttacatatgcttcaaaattctgctcactgataggtcccatctgtggaagctggatgtcagcaaggcttgaaatgagagcttggcttagacctgccagctctttcagcagactttcattgttctgttctatgagtttgttctcctcctctatcgtctttaagttgctctccatagatgtgatctgggtctgaagtttcatcatatctgcttcaattttaaggttggattcattcagttcctttatttcttcatccaaatgcctaatttcttcatcactctctattcccccagttgctttgagcttgatggtcatgagttcttcagaaaccttgccctttttgataacttgtgcattgagaggacatccagataagcttcggtgggtgacaaaaacattatttacatggcccagcccattgcagcctggcaagggacaatgtggtagctcttgtttgttcagtttccaggagagggaggctccattgagaggattctccttctgtctcttggcagccagaggacagccagaagctgtgcggtgtgatgtgtatttacctgatatgtgaccttggccatcacaccctatcacaggacatttcagttcagggtcttctttttcttccttggtaggggtcattttgacaccacctttccttgcacgagggcatccggacaagcttctgtgggaagcatagtttccagtcacgtgccccgagccatcgcagcctggggttggacacttaagctcctgagagttggcagccatgagggattttagagtcttatctgctaaaggacatccagaaacactgcgatgagatgcatagtttcctgtcacgtggccacttccatcacatcctggtgttggacaggtgattagttcctttttgagatctcttgcatgaagcttgggtttagggcttggtatagaggcctctccaggaaactttttttcctctaaattttctagagagctcactgggtctttctctttctcctcctctgtcttcccgtgagttttgctatagttgataggagtgtcccagccctcttggtcacaaagagcctgatagaatgctgcattgaccagaatgctgcttgttttgaatggggaagaggaaggagttggaatagaagtgttagaggaagttaggggtgcagacttgtccaggattcgattttttttcatgcttaagtccaatgtgccattttcatccacttctatttcggctcccttggcatgcagactctgtggcttgttggagaggatgtctgtggcttccctgcagcgggtggaaaggttcaggatggcagcagctgctgctatgtgggtgtcttcactacattgaccgtagctataagagctggcacggccagggctctgggtgtgggcgcctgcactaggcagtcgattaggaaatttcactggatttggaaaatgctttgattcaggaaatggtggtgtttttcgtccttgcactgtttgtatgagagggcgtttaccgaaaacttgggcatcaaaactggcataatcaaatggtacttttccaaacttctcttgttcttttgacactgtggctctgggagaggtgatggcttgtgacgggaaattgaattcaatttgcttcaccaaacttgtcctgtgggcctggtcaggacactgcccagtttggggagaatcaagctgatttttatcctgggacattgccaatttttcagctgcagcaattggacaaccagaaagactcctgtgggtgttgcggttgctgttcacatgaccccttcctgtgcatcccggcgtgggacacttgagcacattttcatgcatggcaagaatttccaggggaacccgcactttgtgggggcaccccgaaaggctgcggtggtgcgggtagagccctgtcacgtgtcccgtgccatcacatccagggatcgggcacttggtctccctcttttcaggccttggtgaatgtttattgttaaagatttgtcttccacccatgtcgataactttggtttgcctcctttcccctgctaggtgctccagcaggaacctatccagctctttgtaggtgttatggaaaacacaacctcgctcagcctgcagagcaattgcctgctccagcaaacttaaattccccttggccttttccaggtcactaccctcttccgtcattactgccaggctctcgctatcttcctcctcaacgtcagggaatgagggctgggcattgccatccaggggttctgcgagagcattctgcgggtctttcctttctgtttcagaatcacacctgttctcacaagggataaatttgtcaccttcagtttttatttcaggaacttccaataggtcttttttatgatctgttaaaacatactttgggactctaggtggtttggtttcttctgagaagttggagccactgtcccagccattttctgcactttcagagttactttcattgtcatcagaggagcagaagggtggctgagaatcatcaatcttgtctcttccatcatcagaatgaatcagaaagcactcgtctgcttcatcgctctctgcttttaaagactggatgccactgtcatttaaattttcacttacagtctgaacagatacatttttttcaaatttccccaagtgcattaaagacttgaccatgagctcttgataacaagagtatctgtcttccttcctactggagttttcttgtgcagttgaaagaagactttcatccataggttttatcatgatttcctctgcggtagagtgaccatgtgtttccaaggggccatcgtcctctgtcctgtcactgcggtcttcttggcagtctgcttttgggctgtagtgtcggggcttcattagcagggatttccttttgttgactggaacccccaaagcctgatcttcagctgttctcttctttgccatggagcaatcataggcaacactttttttctctgaatgacttggttcctttaaaggactctggtgtccctcaccaggtaagtggcctcatgtccacgggcacactgattctgagctcctggattagtgaatccattggcacctcggttcctttagagcgagtacgcagcgttttatcttcagcctctgcatccataaacctataaacagatgtataaagtgatttcctagtacttgtacttgacgtcttttcttactggagcttacatcaggggcaataagcaggtctcttccacatcgccccagtgcacagatctggtaccttcttttaggctgaagaggaagtcctggaattgctctctttttctccaggtaacttgtatgtcaactcagtttgccctgctgtgtcagggggactaaataaatgactttgtcttatttagtgataaatcctgaaattcattctttcttgcagaaaatttctaccgtcctgccttctctaccctttgcagtatatcaaagtgctcagctttttaatcatagatttctgtgtttcttgtaggatttgaccagacattaaatagatgcttcttcaacttaagtcagcaactgtagttccttccctaaaagctactggatctgaactggagagtttccatcactccttagtcttgatatgagcacgcagacacataaaatggaattgtcacaatgcttcagggacactcacaaaattgggggctttttttgtttgtttccaaaacttatatttctctcctccctggtgggctgaacggaaacactaaagctgtttctttgaaaggtagttcccatgatatgac

SEQ ID NO: 18704 - RNA, 5190 nt, Homo sapiens
  source 1..5190: mol_type = other RNA
tgagtgtgtgtgtgtgagtgtgtgtgtatattttgtagcatttgaagttttgtggcaagatttctatcaaattgaatgttgtcttgtttcctatggtgggtgagacccaaggtgccagtgtttgaagtaatcattcagattggagtagcattttttcatgtgttactatattttccattcctttccagtcaacccagtaagataaatgctatttcaggggatatggtatctacaaaatttttcatttggatgtgtttgtatttgctaagtacaaatctacaccaatattgtcacttgtatattgtaccaacatatggcaggaaagcctggctggtcacaccaagtcttatttttcatcttgggatacgagttgccaacgatctgatatgacttgaaaaacaaacagacaaatctgcatcactaaaaaggcttatgtttctttaaaacatttcaaataaataattcatattaacgaaaaccgtccagccaagtcgaatactttgctgattgctatatttaattattgctaacaaattctgagcaggctgttttccagcatcctgtgcttttgtgagtgcggattccccactagtgggcgccatttgtcttcttattccttccgtgcagctcaccttaccgcaaattcatttataaatacaaaaatcagtgaaaggtgggggaagaagtgtgcaataaaaatcaaactcaactatagtgcagtccttagacaaggatttccttcaccctttcctgtttcctcattaaaacccagcaagaaagatgacttgagaatagcatttctatttaaatcctattggaaaataaattaataaacacacttgtaaaaatacggcagacttcaaaatgcagttaaaagataaaaaactctttgattagtaataaataaattataaaaatgtcacatttattttacatatactttacaaaaaaaaaaagagtacaatgaagaaataaaagaaaaacatatgaaaataaataagatctaataattgactgcattgcttttaatccaagaagtctatcatagtttttctttcctttttatatcagctggggaaaataaaattagtgcaatgttgcaaattgtaaatgcagtacggcaacctccacgccttagcagtacatgaacctctaacagatccatctggagtttactgctgttggtaacttctgttgcccggcagcgctgtgatcctacacatggatacccttcactgcctgtttgatactttccagtagagctttgcattccggggaatagtcccgttccagattgctgtacatatctgtgagtgtatttacatatgcttcaaaattctgctcactgataggtcccatctgtggaagctggatgtcagcaaggcttgaaatgagagcttggcttagacctgccagctctttcagcagactttcattgttctgttctatgagtttgttctcctcctctatcgtctttaagttgctctccatagatgtgatctgggtctgaagtttcatcatatctgcttcaattttaaggttggattcattcagttcctttatttcttcatccaaatgcctaatttcttcatcactctctattcccccagttgctttgagcttgatggtcatgagttcttcagaaaccttgccctttttgataacttgtgcattgagaggacatccagataagcttcggtgggtgacaaaaacattatttacatggcccagcccattgcagcctggcaagggacaatgtggtagctcttgtttgttcagtttccaggagagggaggctccattgagaggattctccttctgtctcttggcagccagaggacagccagaagctgtgcggtgtgatgtgtatttacctgatatgtgaccttggccatcacaccctatcacaggacatttcagttcagggtcttctttttcttccttggtaggggtcattttgacaccacctttccttgcacgagggcatccggacaagcttctgtgggaagcatagtttccagtcacgtgccccgagccatcgcagcctggggttggacacttaagctcctgagagttggcagccatgagggattttagagtcttatctgctaaaggacatccagaaacactgcgatgagatgcatagtttcctgtcacgtggccacttccatcacatcctggtgttggacaggtgattagttcctttttgagatctcttgcatgaagcttgggtttagggcttggtatagaggcctctccaggaaactttttttcctctaaattttctagagagctcactgggtctttctctttctcctcctctgtcttcccgtgagttttgctatagttgataggagtgtcccagccctcttggtcacaaagagcctgatagaatgctgcattgaccagaatgctgcttgttttgaatggggaagaggaaggagttggaatagaagtgttagaggaagttaggggtgcagacttgtccaggattcgattttttttcatgcttaagtccaatgtgccattttcatccacttctatttcggctcccttggcatgcagactctgtggcttgttggagaggatgtctgtggcttccctgcagcgggtggaaaggttcaggatggcagcagctgctgctatgtgggtgtcttcactacattgaccgtagctataagagctggcacggccagggctctgggtgtgggcgcctgcactaggcagtcgattaggaaatttcactggatttggaaaatgctttgattcaggaaatggtggtgtttttcgtccttgcactgtttgtatgagagggcgtttaccgaaaacttgggcatcaaaactggcataatcaaatggtacttttccaaacttctcttgttcttttgacactgtggctctgggagaggtgatggcttgtgacgggaaattgaattcaatttgcttcaccaaacttgtcctgtgggcctggtcaggacactgcccagtttggggagaatcaagctgatttttatcctgggacattgccaatttttcagctgcagcaattggacaaccagaaagactcctgtgggtgttgcggttgctgttcacatgaccccttcctgtgcatcccggcgtgggacacttgagcacattttcatgcatggcaagaatttccaggggaacccgcactttgtgggggcaccccgaaaggctgcggtggtgcgggtagagccctgtcacgtgtcccgtgccatcacatccagggatcgggcacttggtctccctcttttcaggccttggtgaatgtttattgttaaagatttgtcttccacccatgtcgataactttggtttgcctcctttcccctgctaggtgctccagcaggaacctatccagctctttgtaggtgttatggaaaacacaacctcgctcagcctgcagagcaattgcctgctccagcaaacttaaattccccttggccttttccaggtcactaccctcttccgtcattactgccaggctctcgctatcttcctcctcaacgtcagggaatgagggctgggcattgccatccaggggttctgcgagagcattctgcgggtctttcctttctgtttcagaatcacacctgttctcacaagggataaatttgtcaccttcagtttttatttcaggaacttccaataggtcttttttatgatctgttaaaacatactttgggactctaggtggtttggtttcttctgagaagttggagccactgtcccagccattttctgcactttcagagttactttcattgtcatcagaggagcagaagggtggctgagaatcatcaatcttgtctcttccatcatcagaatgaatcagaaagcactcgtctgcttcatcgctctctgcttttaaagactggatgccactgtcatttaaattttcacttacagtctgaacagatacatttttttcaaatttccccaagtgcattaaagacttgaccatgagctcttgataacaagagtatctgtcttccttcctactggagttttcttgtgcagttgaaagaagactttcatccataggttttatcatgatttcctctgcggtagagtgaccatgtgtttccaaggggccatcgtcctctgtcctgtcactgcggtcttcttggcagtctgcttttgggctgtagtgtcggggcttcattagcagggatttccttttgttgactggaacccccaaagcctgatcttcagctgttctcttctttgccatggagcaatcataggcaacactttttttctctgaatgacttggttcctttaaaggactctggtgtccctcaccaggtaagtggcctcatgtccacgggcacactgattctgagctcctggattagtgaatccattggcacctcggttcctttagagcgagtacgcagcgttttatcttcagcctctgcatccatctataaacagatgtataaagtgatttcctagtacttgtacttgacgtcttttcttactggagcttacatcaggggcaataagcaggtctcttccacatcgccccagtgcacagatctggtaccttcttttaggctgaagaggaagtcctggaattgctctctttttctccaggtaacttgtatgtcaactcagtttgccctgctgtgtcagggggactaaataaatgactttgtcttatttagtgataaatcctgaaattcattctttcttgcagaaaatttctaccgtcctgccttctctaccctttgcagtatatcaaagtgctcagctttttaatcatagatttctgtgtttcttgtaggatttgaccagacattaaatagatgcttcttcaacttaagtcagcaactgtagttccttccctaaaagctactggatctgaactggagagtttccatcactccttagtcttgatatgagcacgcagacacataaaatggaattgtcacaatgcttcagggacactcacaaaattgggggctctttacctggcgaacgtctacaggtgtgtcgaaagttatcttttcctggatgtgttccaaaatgctcttatgctatttctcttaggatttctccacgctgccccattcagaaattttattattttctctagtattcccctgaggtcacattcagttaaaaacatcctgcccttctccctacaaaaaggttccatagaatc

SEQ ID NO: 18705 - RNA, 5089 nt, Homo sapiens
  source 1..5089: mol_type = other RNA
tgagtgtgtgtgtgtgagtgtgtgtgtatattttgtagcatttgaagttttgtggcaagatttctatcaaattgaatgttgtcttgtttcctatggtgggtgagacccaaggtgccagtgtttgaagtaatcattcagattggagtagcattttttcatgtgttactatattttccattcctttccagtcaacccagtaagataaatgctatttcaggggatatggtatctacaaaatttttcatttggatgtgtttgtatttgctaagtacaaatctacaccaatattgtcacttgtatattgtaccaacatatggcaggaaagcctggctggtcacaccaagtcttatttttcatcttgggatacgagttgccaacgatctgatatgacttgaaaaacaaacagacaaatctgcatcactaaaaaggcttatgtttctttaaaacatttcaaataaataattcatattaacgaaaaccgtccagccaagtcgaatactttgctgattgctatatttaattattgctaacaaattctgagcaggctgttttccagcatcctgtgcttttgtgagtgcggattccccactagtgggcgccatttgtcttcttattccttccgtgcagctcaccttaccgcaaattcatttataaatacaaaaatcagtgaaaggtgggggaagaagtgtgcaataaaaatcaaactcaactatagtgcagtccttagacaaggatttccttcaccctttcctgtttcctcattaaaacccagcaagaaagatgacttgagaatagcatttctatttaaatcctattggaaaataaattaataaacacacttgtaaaaatacggcagacttcaaaatgcagttaaaagataaaaaactctttgattagtaataaataaattataaaaatgtcacatttattttacatatactttacaaaaaaaaaaagagtacaatgaagaaataaaagaaaaacatatgaaaataaataagatctaataattgactgcattgcttttaatccaagaagtctatcatagtttttctttcctttttatatcagctggggaaaataaaattagtgcaatgttgcaaattgtaaatgcagtacggcaacctccacgccttagcagtacatgaacctctaacagatccatctggagtttactgctgttggtaacttctgttgcccggcagcgctgtgatcctacacatggatacccttcactgcctgtttgatactttccagtagagctttgcattccggggaatagtcccgttccagattgctgtacatatctgtgagtgtatttacatatgcttcaaaattctgctcactgataggtcccatctgtggaagctggatgtcagcaaggcttgaaatgagagcttggcttagacctgccagctctttcagcagactttcattgttctgttctatgagtttgttctcctcctctatcgtctttaagttgctctccatagatgtgatctgggtctgaagtttcatcatatctgcttcaattttaaggttggattcattcagttcctttatttcttcatccaaatgcctaatttcttcatcactctctattcccccagttgctttgagcttgatggtcatgagttcttcagaaaccttgccctttttgataacttgtgcattgagaggacatccagataagcttcggtgggtgacaaaaacattatttacatggcccagcccattgcagcctggcaagggacaatgtggtagctcttgtttgttcagtttccaggagagggaggctccattgagaggattctccttctgtctcttggcagccagaggacagccagaagctgtgcggtgtgatgtgtatttacctgatatgtgaccttggccatcacaccctatcacaggacatttcagttcagggtcttctttttcttccttggtaggggtcattttgacaccacctttccttgcacgagggcatccggacaagcttctgtgggaagcatagtttccagtcacgtgccccgagccatcgcagcctggggttggacacttaagctcctgagagttggcagccatgagggattttagagtcttatctgctaaaggacatccagaaacactgcgatgagatgcatagtttcctgtcacgtggccacttccatcacatcctggtgttggacaggtgattagttcctttttgagatctcttgcatgaagcttgggtttagggcttggtatagaggcctctccaggaaactttttttcctctaaattttctagagagctcactgggtctttctctttctcctcctctgtcttcccgtgagttttgctatagttgataggagtgtcccagccctcttggtcacaaagagcctgatagaatgctgcattgaccagaatgctgcttgttttgaatggggaagaggaaggagttggaatagaagtgttagaggaagttaggggtgcagacttgtccaggattcgattttttttcatgcttaagtccaatgtgccattttcatccacttctatttcggctcccttggcatgcagactctgtggcttgttggagaggatgtctgtggcttccctgcagcgggtggaaaggttcaggatggcagcagctgctgctatgtgggtgtcttcactacattgaccgtagctataagagctggcacggccagggctctgggtgtgggcgcctgcactaggcagtcgattaggaaatttcactggatttggaaaatgctttgattcaggaaatggtggtgtttttcgtccttgcactgtttgtatgagagggcgtttaccgaaaacttgggcatcaaaactggcataatcaaatggtacttttccaaacttctcttgttcttttgacactgtggctctgggagaggtgatggcttgtgacgggaaattgaattcaatttgcttcaccaaacttgtcctgtgggcctggtcaggacactgcccagtttggggagaatcaagctgatttttatcctgggacattgccaatttttcagctgcagcaattggacaaccagaaagactcctgtgggtgttgcggttgctgttcacatgaccccttcctgtgcatcccggcgtgggacacttgagcacattttcatgcatggcaagaatttccaggggaacccgcactttgtgggggcaccccgaaaggctgcggtggtgcgggtagagccctgtcacgtgtcccgtgccatcacatccagggatcgggcacttggtctccctcttttcaggccttggtgaatgtttattgttaaagatttgtcttccacccatgtcgataactttggtttgcctcctttcccctgctaggtgctccagcaggaacctatccagctctttgtaggtgttatggaaaacacaacctcgctcagcctgcagagcaattgcctgctccagcaaacttaaattccccttggccttttccaggtcactaccctcttccgtcattactgccaggctctcgctatcttcctcctcaacgtcagggaatgagggctgggcattgccatccaggggttctgcgagagcattctgcgggtctttcctttctgtttcagaatcacacctgttctcacaagggataaatttgtcaccttcagtttttatttcaggaacttccaataggtcttttttatgatctgttaaaacatactttgggactctaggtggtttggtttcttctgagaagttggagccactgtcccagccattttctgcactttcagagttactttcattgtcatcagaggagcagaagggtggctgagaatcatcaatcttgtctcttccatcatcagaatgaatcagaaagcactcgtctgcttcatcgctctctgcttttaaagactggatgccactgtcatttaaattttcacttacagtctgaacagatacatttttttcaaatttccccaagtgcattaaagacttgaccatgagctcttgataacaagagtatctgtcttccttcctactggagttttcttgtgcagttgaaagaagactttcatccataggttttatcatgatttcctctgcggtagagtgaccatgtgtttccaaggggccatcgtcctctgtcctgtcactgcggtcttcttggcagtctgcttttgggctgtagtgtcggggcttcattagcagggatttccttttgttgactggaacccccaaagcctgatcttcagctgttctcttctttgccatggagcaatcataggcaacactttttttctctgaatgacttggttcctttaaaggactctggtgtccctcaccaggtaagtggcctcatgtccacgggcacactgattctgagctcctggattagtgaatccattggcacctcggttcctttagagcgagtacgcagcgttttatcttcagcctctgcatccatctataaacagatgtataaagtgatttcctagtacttgtacttgacgtcttttcttactggagcttacatcaggggcaataagcaggtctcttccacatcgccccagtgcacagatctggtaccttcttttaggctgaagaggaagtcctggaattgctctctttttctccaggtaacttgtatgtcaactcagtttgccctgctgtgtcagggggactaaataaatgactttgtcttatttagtgataaatcctgaaattcattctttcttgcagaaaatttctaccgtcctgccttctctaccctttgcagtatatcaaagtgctcagctttttaatcatagatttctgtgtttcttgtaggatttgaccagacattaaatagatgcttcttcaacttaagtcagcaactgtagttccttccctaaaagctactggatctgaactggagagtttccatcactccttagtcttgatatgagcacgcagacacataaaatggaattgtcacaatgcttcagggacactcacaaaattgggggctttttttgtttgtttccaaaacttatatttctctcctccctggtgggctgaacggaaacactaaagctgtttctttgaaaggtagttcccatgatatgac

SEQ ID NO: 18706 - RNA, 5010 nt, Homo sapiens
  source 1..5010: mol_type = other RNA
tgagtgtgtgtgtgtgagtgtgtgtgtatattttgtagcatttgaagttttgtggcaagatttctatcaaattgaatgttgtcttgtttcctatggtgggtgagacccaaggtgccagtgtttgaagtaatcattcagattggagtagcattttttcatgtgttactatattttccattcctttccagtcaacccagtaagataaatgctatttcaggggatatggtatctacaaaatttttcatttggatgtgtttgtatttgctaagtacaaatctacaccaatattgtcacttgtatattgtaccaacatatggcaggaaagcctggctggtcacaccaagtcttatttttcatcttgggatacgagttgccaacgatctgatatgacttgaaaaacaaacagacaaatctgcatcactaaaaaggcttatgtttctttaaaacatttcaaataaataattcatattaacgaaaaccgtccagccaagtcgaatactttgctgattgctatatttaattattgctaacaaattctgagcaggctgttttccagcatcctgtgcttttgtgagtgcggattccccactagtgggcgccatttgtcttcttattccttccgtgcagctcaccttaccgcaaattcatttataaatacaaaaatcagtgaaaggtgggggaagaagtgtgcaataaaaatcaaactcaactatagtgcagtccttagacaaggatttccttcaccctttcctgtttcctcattaaaacccagcaagaaagatgacttgagaatagcatttctatttaaatcctattggaaaataaattaataaacacacttgtaaaaatacggcagacttcaaaatgcagttaaaagataaaaaactctttgattagtaataaataaattataaaaatgtcacatttattttacatatactttacaaaaaaaaaaagagtacaatgaagaaataaaagaaaaacatatgaaaataaataagatctaataattgactgcattgcttttaatccaagaagtctatcatagtttttctttcctttttatatcagctggggaaaataaaattagtgcaatgttgcaaattgtaaatgcagtacggcaacctccacgccttagcagtacatgaacctctaacagatccatctggagtttactgctgttggtaacttctgttgcccggcagcgctgtgatcctacacatggatacccttcactgcctgtttgatactttccagtagagctttgcattccggggaatagtcccgttccagattgctgtacatatctgtgagtgtatttacatatgcttcaaaattctgctcactgataggtcccatctgtggaagctggatgtcagcaaggcttgaaatgagagcttggcttagacctgccagctctttcagcagactttcattgttctgttctatgagtttgttctcctcctctatcgtctttaagttgctctccatagatgtgatctgggtctgaagtttcatcatatctgcttcaattttaaggttggattcattcagttcctttatttcttcatccaaatgcctaatttcttcatcactctctattcccccagttgctttgagcttgatggtcatgagttcttcagaaaccttgccctttttgataacttgtgcattgagaggacatccagataagcttcggtgggtgacaaaaacattatttacatggcccagcccattgcagcctggcaagggacaatgtggtagctcttgtttgttcagtttccaggagagggaggctccattgagaggattctccttctgtctcttggcagccagaggacagccagaagctgtgcggtgtgatgtgtatttacctgatatgtgaccttggccatcacaccctatcacaggacatttcagttcagggtcttctttttcttccttggtaggggtcattttgacaccacctttccttgcacgagggcatccggacaagcttctgtgggaagcatagtttccagtcacgtgccccgagccatcgcagcctggggttggacacttaagctcctgagagttggcagccatgagggattttagagtcttatctgctaaaggacatccagaaacactgcgatgagatgcatagtttcctgtcacgtggccacttccatcacatcctggtgttggacaggtgattagttcctttttgagatctcttgcatgaagcttgggtttagggcttggtatagaggcctctccaggaaactttttttcctctaaattttctagagagctcactgggtctttctctttctcctcctctgtcttcccgtgagttttgctatagttgataggagtgtcccagccctcttggtcacaaagagcctgatagaatgctgcattgaccagaatgctgcttgttttgaatggggaagaggaaggagttggaatagaagtgttagaggaagttaggggtgcagacttgtccaggattcgattttttttcatgcttaagtccaatgtgccattttcatccacttctatttcggctcccttggcatgcagactctgtggcttgttggagaggatgtctgtggcttccctgcagcgggtggaaaggttcaggatggcagcagctgctgctatgtgggtgtcttcactacattgaccgtagctataagagctggcacggccagggctctgggtgtgggcgcctgcactaggcagtcgattaggaaatttcactggatttggaaaatgctttgattcaggaaatggtggtgtttttcgtccttgcactgtttgtatgagagggcgtttaccgaaaacttgggcatcaaaactggcataatcaaatggtacttttccaaacttctcttgttcttttgacactgtggctctgggagaggtgatggcttgtgacgggaaattgaattcaatttgcttcaccaaacttgtcctgtgggcctggtcaggacactgcccagtttggggagaatcaagctgatttttatcctgggacattgccaatttttcagctgcagcaattggacaaccagaaagactcctgtgggtgttgcggttgctgttcacatgaccccttcctgtgcatcccggcgtgggacacttgagcacattttcatgcatggcaagaatttccaggggaacccgcactttgtgggggcaccccgaaaggctgcggtggtgcgggtagagccctgtcacgtgtcccgtgccatcacatccagggatcgggcacttggtctccctcttttcaggccttggtgaatgtttattgttaaagatttgtcttccacccatgtcgataactttggtttgcctcctttcccctgctaggtgctccagcaggaacctatccagctctttgtaggtgttatggaaaacacaacctcgctcagcctgcagagcaattgcctgctccagcaaacttaaattccccttggccttttccaggtcactaccctcttccgtcattactgccaggctctcgctatcttcctcctcaacgtcagggaatgagggctgggcattgccatccaggggttctgcgagagcattctgcgggtctttcctttctgtttcagaatcacacctgttctcacaagggataaatttgtcaccttcagtttttatttcaggaacttccaataggtcttttttatgatctgttaaaacatactttgggactctaggtggtttggtttcttctgagaagttggagccactgtcccagccattttctgcactttcagagttactttcattgtcatcagaggagcagaagggtggctgagaatcatcaatcttgtctcttccatcatcagaatgaatcagaaagcactcgtctgcttcatcgctctctgcttttaaagactggatgccactgtcatttaaattttcacttacagtctgaacagatacatttttttcaaatttccccaagtgcattaaagacttgaccatgagctcttgataacaagagtatctgtcttccttcctactggagttttcttgtgcagttgaaagaagactttcatccataggttttatcatgatttcctctgcggtagagtgaccatgtgtttccaaggggccatcgtcctctgtcctgtcactgcggtcttcttggcagtctgcttttgggctgtagtgtcggggcttcattagcagggatttccttttgttgactggaacccccaaagcctgatcttcagctgttctcttctttgccatggagcaatcataggcaacactttttttctctgaatgacttggttcctttaaaggactctggtgtccctcaccaggtaagtggcctcatgtccacgggcacactgattctgagctcctggattagtgaatccattggcacctcggttcctttagagcgagtacgcagcgttttatcttcagcctctgcatccatctataaacagatgtataaagtgatttcctagtacttgtacttgacgtcttttcttactggagcttacatcaggggcaataagcaggtctcttccacatcgccccagtgcacagatctggtaccttcttttaggctgaagaggaagtcctggaattgctctctttttctccaggtaacttgtatgtcaactcagtttgccctgctgtgtcagggggactaaataaatgactttgtcttatttagtgataaatcctgaaattcattctttcttgcagaaaatttctaccgtcctgccttctctaccctttgcagtatatcaaagtgctcagctttttaatcatagatttctgtgtttcttgtaggatttgaccagacattaaatagatgcttcttcaacttaagtcagcaactgtagttccttccctaaaagctactggatctgaactggagagtttccatcactcttttttgtttgtttccaaaacttatatttctctcctccctggtgggctgaacggaaacactaaagctgtttctttgaaaggtagttcccatgatatgac

SEQ ID NO: 18707 - RNA, 5000 nt, Homo sapiens
  source 1..5000: mol_type = other RNA
tgagtgtgtgtgtgtgagtgtgtgtgtatattttgtagcatttgaagttttgtggcaagatttctatcaaattgaatgttgtcttgtttcctatggtgggtgagacccaaggtgccagtgtttgaagtaatcattcagattggagtagcattttttcatgtgttactatattttccattcctttccagtcaacccagtaagataaatgctatttcaggggatatggtatctacaaaatttttcatttggatgtgtttgtatttgctaagtacaaatctacaccaatattgtcacttgtatattgtaccaacatatggcaggaaagcctggctggtcacaccaagtcttatttttcatcttgggatacgagttgccaacgatctgatatgacttgaaaaacaaacagacaaatctgcatcactaaaaaggcttatgtttctttaaaacatttcaaataaataattcatattaacgaaaaccgtccagccaagtcgaatactttgctgattgctatatttaattattgctaacaaattctgagcaggctgttttccagcatcctgtgcttttgtgagtgcggattccccactagtgggcgccatttgtcttcttattccttccgtgcagctcaccttaccgcaaattcatttataaatacaaaaatcagtgaaaggtgggggaagaagtgtgcaataaaaatcaaactcaactatagtgcagtccttagacaaggatttccttcaccctttcctgtttcctcattaaaacccagcaagaaagatgacttgagaatagcatttctatttaaatcctattggaaaataaattaataaacacacttgtaaaaatacggcagacttcaaaatgcagttaaaagataaaaaactctttgattagtaataaataaattataaaaatgtcacatttattttacatatactttacaaaaaaaaaaagagtacaatgaagaaataaaagaaaaacatatgaaaataaataagatctaataattgactgcattgcttttaatccaagaagtctatcatagtttttctttcctttttatatcagctggggaaaataaaattagtgcaatgttgcaaattgtaaatgcagtacggcaacctccacgccttagcagtacatgaacctctaacagatccatctggagtttactgctgttggtaacttctgttgcccggcagcgctgtgatcctacacatggatacccttcactgcctgtttgatactttccagtagagctttgcattccggggaatagtcccgttccagattgctgtacatatctgtgagtgtatttacatatgcttcaaaattctgctcactgataggtcccatctgtggaagctggatgtcagcaaggcttgaaatgagagcttggcttagacctgccagctctttcagcagactttcattgttctgttctatgagtttgttctcctcctctatcgtctttaagttgctctccatagatgtgatctgggtctgaagtttcatcatatctgcttcaattttaaggttggattcattcagttcctttatttcttcatccaaatgcctaatttcttcatcactctctattcccccagttgctttgagcttgatggtcatgagttcttcagaaaccttgccctttttgataacttgtgcattgagaggacatccagataagcttcggtgggtgacaaaaacattatttacatggcccagcccattgcagcctggcaagggacaatgtggtagctcttgtttgttcagtttccaggagagggaggctccattgagaggattctccttctgtctcttggcagccagaggacagccagaagctgtgcggtgtgatgtgtatttacctgatatgtgaccttggccatcacaccctatcacaggacatttcagttcagggtcttctttttcttccttggtaggggtcattttgacaccacctttccttgcacgagggcatccggacaagcttctgtgggaagcatagtttccagtcacgtgccccgagccatcgcagcctggggttggacacttaagctcctgagagttggcagccatgagggattttagagtcttatctgctaaaggacatccagaaacactgcgatgagatgcatagtttcctgtcacgtggccacttccatcacatcctggtgttggacaggtgattagttcctttttgagatctcttgcatgaagcttgggtttagggcttggtatagaggcctctccaggaaactttttttcctctaaattttctagagagctcactgggtctttctctttctcctcctctgtcttcccgtgagttttgctatagttgataggagtgtcccagccctcttggtcacaaagagcctgatagaatgctgcattgaccagaatgctgcttgttttgaatggggaagaggaaggagttggaatagaagtgttagaggaagttaggggtgcagacttgtccaggattcgattttttttcatgcttaagtccaatgtgccattttcatccacttctatttcggctcccttggcatgcagactctgtggcttgttggagaggatgtctgtggcttccctgcagcgggtggaaaggttcaggatggcagcagctgctgctatgtgggtgtcttcactacattgaccgtagctataagagctggcacggccagggctctgggtgtgggcgcctgcactaggcagtcgattaggaaatttcactggatttggaaaatgctttgattcaggaaatggtggtgtttttcgtccttgcactgtttgtatgagagggcgtttaccgaaaacttgggcatcaaaactggcataatcaaatggtacttttccaaacttctcttgttcttttgacactgtggctctgggagaggtgatggcttgtgacgggaaattgaattcaatttgcttcaccaaacttgtcctgtgggcctggtcaggacactgcccagtttggggagaatcaagctgatttttatcctgggacattgccaatttttcagctgcagcaattggacaaccagaaagactcctgtgggtgttgcggttgctgttcacatgaccccttcctgtgcatcccggcgtgggacacttgagcacattttcatgcatggcaagaatttccaggggaacccgcactttgtgggggcaccccgaaaggctgcggtggtgcgggtagagccctgtcacgtgtcccgtgccatcacatccagggatcgggcacttggtctccctcttttcaggccttggtgaatgtttattgttaaagatttgtcttccacccatgtcgataactttggtttgcctcctttcccctgctaggtgctccagcaggaacctatccagctctttgtaggtgttatggaaaacacaacctcgctcagcctgcagagcaattgcctgctccagcaaacttaaattccccttggccttttccaggtcactaccctcttccgtcattactgccaggctctcgctatcttcctcctcaacgtcagggaatgagggctgggcattgccatccaggggttctgcgagagcattctgcgggtctttcctttctgtttcagaatcacacctgttctcacaagggataaatttgtcaccttcagtttttatttcaggaacttccaataggtcttttttatgatctgttaaaacatactttgggactctaggtggtttggtttcttctgagaagttggagccactgtcccagccattttctgcactttcagagttactttcattgtcatcagaggagcagaagggtggctgagaatcatcaatcttgtctcttccatcatcagaatgaatcagaaagcactcgtctgcttcatcgctctctgcttttaaagactggatgccactgtcatttaaattttcacttacagtctgaacagatacatttttttcaaatttccccaagtgcattaaagacttgaccatgagctcttgataacaagagtatctgtcttccttcctactggagttttcttgtgcagttgaaagaagactttcatccataggttttatcatgatttcctctgcggtagagtgaccatgtgtttccaaggggccatcgtcctctgtcctgtcactgcggtcttcttggcagtctgcttttgggctgtagtgtcggggcttcattagcagggatttccttttgttgactggaacccccaaagcctgatcttcagctgttctcttctttgccatggagcaatcataggcaacactttttttctctgaatgacttggttcctttaaaggactctggtgtccctcaccaggtaagtggcctcatgtccacgggcacactgattctgagctcctggattagtgaatccattggcacctcggttcctttagagcgagtacgcagcgttttatcttcagcctctgcatccatctctctttttctccaggtaacttgtatgtcaactcagtttgccctgctgtgtcagggggactaaataaatgactttgtcttatttagtgataaatcctgaaattcattctttcttgcagaaaatttctaccgtcctgccttctctaccctttgcagtatatcaaagtgctcagctttttaatcatagatttctgtgtttcttgtaggatttgaccagacattaaatagatgcttcttcaacttaagtcagcaactgtagttccttccctaaaagctactggatctgaactggagagtttccatcactccttagtcttgatatgagcacgcagacacataaaatggaattgtcacaatgcttcagggacactcacaaaattgggggctctgaatgtcttgtaacaatatcatcctctcttgaactaaacatcctctgaatacacaaatctaaggcagacagacatttcagcaaggcaaataagactttctggcaacttcctgttgccatatttctctcaaaggatcctgcaatgttacacttcaatcctgcaaa

SEQ ID NO: 18708 - RNA, 5034 nt, Homo sapiens
  source 1..5034: mol_type = other RNA
tgagtgtgtgtgtgtgagtgtgtgtgtatattttgtagcatttgaagttttgtggcaagatttctatcaaattgaatgttgtcttgtttcctatggtgggtgagacccaaggtgccagtgtttgaagtaatcattcagattggagtagcattttttcatgtgttactatattttccattcctttccagtcaacccagtaagataaatgctatttcaggggatatggtatctacaaaatttttcatttggatgtgtttgtatttgctaagtacaaatctacaccaatattgtcacttgtatattgtaccaacatatggcaggaaagcctggctggtcacaccaagtcttatttttcatcttgggatacgagttgccaacgatctgatatgacttgaaaaacaaacagacaaatctgcatcactaaaaaggcttatgtttctttaaaacatttcaaataaataattcatattaacgaaaaccgtccagccaagtcgaatactttgctgattgctatatttaattattgctaacaaattctgagcaggctgttttccagcatcctgtgcttttgtgagtgcggattccccactagtgggcgccatttgtcttcttattccttccgtgcagctcaccttaccgcaaattcatttataaatacaaaaatcagtgaaaggtgggggaagaagtgtgcaataaaaatcaaactcaactatagtgcagtccttagacaaggatttccttcaccctttcctgtttcctcattaaaacccagcaagaaagatgacttgagaatagcatttctatttaaatcctattggaaaataaattaataaacacacttgtaaaaatacggcagacttcaaaatgcagttaaaagataaaaaactctttgattagtaataaataaattataaaaatgtcacatttattttacatatactttacaaaaaaaaaaagagtacaatgaagaaataaaagaaaaacatatgaaaataaataagatctaataattgactgcattgcttttaatccaagaagtctatcatagtttttctttcctttttatatcagctggggaaaataaaattagtgcaatgttgcaaattgtaaatgcagtacggcaacctccacgccttagcagtacatgaacctctaacagatccatctggagtttactgctgttggtaacttctgttgcccggcagcgctgtgatcctacacatggatacccttcactgcctgtttgatactttccagtagagctttgcattccggggaatagtcccgttccagattgctgtacatatctgtgagtgtatttacatatgcttcaaaattctgctcactgataggtcccatctgtggaagctggatgtcagcaaggcttgaaatgagagcttggcttagacctgccagctctttcagcagactttcattgttctgttctatgagtttgttctcctcctctatcgtctttaagttgctctccatagatgtgatctgggtctgaagtttcatcatatctgcttcaattttaaggttggattcattcagttcctttatttcttcatccaaatgcctaatttcttcatcactctctattcccccagttgctttgagcttgatggtcatgagttcttcagaaaccttgccctttttgataacttgtgcattgagaggacatccagataagcttcggtgggtgacaaaaacattatttacatggcccagcccattgcagcctggcaagggacaatgtggtagctcttgtttgttcagtttccaggagagggaggctccattgagaggattctccttctgtctcttggcagccagaggacagccagaagctgtgcggtgtgatgtgtatttacctgatatgtgaccttggccatcacaccctatcacaggacatttcagttcagggtcttctttttcttccttggtaggggtcattttgacaccacctttccttgcacgagggcatccggacaagcttctgtgggaagcatagtttccagtcacgtgccccgagccatcgcagcctggggttggacacttaagctcctgagagttggcagccatgagggattttagagtcttatctgctaaaggacatccagaaacactgcgatgagatgcatagtttcctgtcacgtggccacttccatcacatcctggtgttggacaggtgattagttcctttttgagatctcttgcatgaagcttgggtttagggcttggtatagaggcctctccaggaaactttttttcctctaaattttctagagagctcactgggtctttctctttctcctcctctgtcttcccgtgagttttgctatagttgataggagtgtcccagccctcttggtcacaaagagcctgatagaatgctgcattgaccagaatgctgcttgttttgaatggggaagaggaaggagttggaatagaagtgttagaggaagttaggggtgcagacttgtccaggattcgattttttttcatgcttaagtccaatgtgccattttcatccacttctatttcggctcccttggcatgcagactctgtggcttgttggagaggatgtctgtggcttccctgcagcgggtggaaaggttcaggatggcagcagctgctgctatgtgggtgtcttcactacattgaccgtagctataagagctggcacggccagggctctgggtgtgggcgcctgcactaggcagtcgattaggaaatttcactggatttggaaaatgctttgattcaggaaatggtggtgtttttcgtccttgcactgtttgtatgagagggcgtttaccgaaaacttgggcatcaaaactggcataatcaaatggtacttttccaaacttctcttgttcttttgacactgtggctctgggagaggtgatggcttgtgacgggaaattgaattcaatttgcttcaccaaacttgtcctgtgggcctggtcaggacactgcccagtttggggagaatcaagctgatttttatcctgggacattgccaatttttcagctgcagcaattggacaaccagaaagactcctgtgggtgttgcggttgctgttcacatgaccccttcctgtgcatcccggcgtgggacacttgagcacattttcatgcatggcaagaatttccaggggaacccgcactttgtgggggcaccccgaaaggctgcggtggtgcgggtagagccctgtcacgtgtcccgtgccatcacatccagggatcgggcacttggtctccctcttttcaggccttggtgaatgtttattgttaaagatttgtcttccacccatgtcgataactttggtttgcctcctttcccctgctaggtgctccagcaggaacctatccagctctttgtaggtgttatggaaaacacaacctcgctcagcctgcagagcaattgcctgctccagcaaacttaaattccccttggccttttccaggtcactaccctcttccgtcattactgccaggctctcgctatcttcctcctcaacgtcagggaatgagggctgggcattgccatccaggggttctgcgagagcattctgcgggtctttcctttctgtttcagaatcacacctgttctcacaagggataaatttgtcaccttcagtttttatttcaggaacttccaataggtcttttttatgatctgttaaaacatactttgggactctaggtggtttggtttcttctgagaagttggagccactgtcccagccattttctgcactttcagagttactttcattgtcatcagaggagcagaagggtggctgagaatcatcaatcttgtctcttccatcatcagaatgaatcagaaagcactcgtctgcttcatcgctctctgcttttaaagactggatgccactgtcatttaaattttcacttacagtctgaacagatacatttttttcaaatttccccaagtgcattaaagacttgaccatgagctcttgataacaagagtatctgtcttccttcctactggagttttcttgtgcagttgaaagaagactttcatccataggttttatcatgatttcctctgcggtagagtgaccatgtgtttccaaggggccatcgtcctctgtcctgtcactgcggtcttcttggcagtctgcttttgggctgtagtgtcggggcttcattagcagggatttccttttgttgactggaacccccaaagcctgatcttcagctgttctcttctttgccatggagcaatcataggcaacactttttttctctgaatgacttggttcctttaaaggactctggtgtccctcaccaggtaagtggcctcatgtccacgggcacactgattctgagctcctggattagtgaatccattggcacctcggttcctttagagcgagtacgcagcgttttatcttcagcctctgcatccatctctctttttctccaggtaacttgtatgtcaactcagtttgccctgctgtgtcagggggactaaataaatgactttgtcttatttagtgataaatcctgaaattcattctttcttgcagaaaatttctaccgtcctgccttctctaccctttgcagtatatcaaagtgctcagctttttaatcatagatttctgtgtttcttgtaggatttgaccagacattaaatagatgcttcttcaacttaagtcagcaactgtagttccttccctaaaagctactggatctgaactggagagtttccatcactccttagtcttgatatgagcacgcagacacataaaatggaattgtcacaatgcttcagggacactcacaaaattgggggctctttacctggcgaacgtctacaggtgtgtcgaaagttatcttttcctggatgtgttccaaaatgctcttatgctatttctcttaggatttctccacgctgccccattcagaaattttattattttctctagtattcccctgaggtcacattcagttaaaaacatcctgcccttctccctacaaaaaggttccatagaatc

SEQ ID NO: 18709 - RNA, 4827 nt, Homo sapiens
  source 1..4827: mol_type = other RNA
tgagtgtgtgtgtgtgagtgtgtgtgtatattttgtagcatttgaagttttgtggcaagatttctatcaaattgaatgttgtcttgtttcctatggtgggtgagacccaaggtgccagtgtttgaagtaatcattcagattggagtagcattttttcatgtgttactatattttccattcctttccagtcaacccagtaagataaatgctatttcaggggatatggtatctacaaaatttttcatttggatgtgtttgtatttgctaagtacaaatctacaccaatattgtcacttgtatattgtaccaacatatggcaggaaagcctggctggtcacaccaagtcttatttttcatcttgggatacgagttgccaacgatctgatatgacttgaaaaacaaacagacaaatctgcatcactaaaaaggcttatgtttctttaaaacatttcaaataaataattcatattaacgaaaaccgtccagccaagtcgaatactttgctgattgctatatttaattattgctaacaaattctgagcaggctgttttccagcatcctgtgcttttgtgagtgcggattccccactagtgggcgccatttgtcttcttattccttccgtgcagctcaccttaccgcaaattcatttataaatacaaaaatcagtgaaaggtgggggaagaagtgtgcaataaaaatcaaactcaactatagtgcagtccttagacaaggatttccttcaccctttcctgtttcctcattaaaacccagcaagaaagatgacttgagaatagcatttctatttaaatcctattggaaaataaattaataaacacacttgtaaaaatacggcagacttcaaaatgcagttaaaagataaaaaactctttgattagtaataaataaattataaaaatgtcacatttattttacatatactttacaaaaaaaaaaagagtacaatgaagaaataaaagaaaaacatatgaaaataaataagatctaataattgactgcattgcttttaatccaagaagtctatcatagtttttctttcctttttatatcagctggggaaaataaaattagtgcaatgttgcaaattgtaaatgcagtacggcaacctccacgccttagcagtacatgaacctctaacagatccatctggagtttactgctgttggtaacttctgttgcccggcagcgctgtgatcctacacatggatacccttcactgcctgtttgatactttccagtagagctttgcattccggggaatagtcccgttccagattgctgtacatatctgtgagtgtatttacatatgcttcaaaattctgctcactgataggtcccatctgtggaagctggatgtcagcaaggcttgaaatgagagcttggcttagacctgccagctctttcagcagactttcattgttctgttctatgagtttgttctcctcctctatcgtctttaagttgctctccatagatgtgatctgggtctgaagtttcatcatatctgcttcaattttaaggttggattcattcagttcctttatttcttcatccaaatgcctaatttcttcatcactctctattcccccagttgctttgagcttgatggtcatgagttcttcagaaaccttgccctttttgataacttgtgcattgagaggacatccagataagcttcggtgggtgacaaaaacattatttacatggcccagcccattgcagcctggcaagggacaatgtggtagctcttgtttgttcagtttccaggagagggaggctccattgagaggattctccttctgtctcttggcagccagaggacagccagaagctgtgcggtgtgatgtgtatttacctgatatgtgaccttggccatcacaccctatcacaggacatttcagttcagggtcttctttttcttccttggtaggggtcattttgacaccacctttccttgcacgagggcatccggacaagcttctgtgggaagcatagtttccagtcacgtgccccgagccatcgcagcctggggttggacacttaagctcctgagagttggcagccatgagggattttagagtcttatctgctaaaggacatccagaaacactgcgatgagatgcatagtttcctgtcacgtggccacttccatcacatcctggtgttggacaggtgattagttcctttttgagatctcttgcatgaagcttgggtttagggcttggtatagaggcctctccaggaaactttttttcctctaaattttctagagagctcactgggtctttctctttctcctcctctgtcttcccgtgagttttgctatagttgataggagtgtcccagccctcttggtcacaaagagcctgatagaatgctgcattgaccagaatgctgcttgttttgaatggggaagaggaaggagttggaatagaagtgttagaggaagttaggggtgcagacttgtccaggattcgattttttttcatgcttaagtccaatgtgccattttcatccacttctatttcggctcccttggcatgcagactctgtggcttgttggagaggatgtctgtggcttccctgcagcgggtggaaaggttcaggatggcagcagctgctgctatgtgggtgtcttcactacattgaccgtagctataagagctggcacggccagggctctgggtgtgggcgcctgcactaggcagtcgattaggaaatttcactggatttggaaaatgctttgattcaggaaatggtggtgtttttcgtccttgcactgtttgtatgagagggcgtttaccgaaaacttgggcatcaaaactggcataatcaaatggtacttttccaaacttctcttgttcttttgacactgtggctctgggagaggtgatggcttgtgacgggaaattgaattcaatttgcttcaccaaacttgtcctgtgggcctggtcaggacactgcccagtttggggagaatcaagctgatttttatcctgggacattgccaatttttcagctgcagcaattggacaaccagaaagactcctgtgggtgttgcggttgctgttcacatgaccccttcctgtgcatcccggcgtgggacacttgagcacattttcatgcatggcaagaatttccaggggaacccgcactttgtgggggcaccccgaaaggctgcggtggtgcgggtagagccctgtcacgtgtcccgtgccatcacatccagggatcgggcacttggtctccctcttttcaggccttggtgaatgtttattgttaaagatttgtcttccacccatgtcgataactttggtttgcctcctttcccctgctaggtgctccagcaggaacctatccagctctttgtaggtgttatggaaaacacaacctcgctcagcctgcagagcaattgcctgctccagcaaacttaaattccccttggccttttccaggtcactaccctcttccgtcattactgccaggctctcgctatcttcctcctcaacgtcagggaatgagggctgggcattgccatccaggggttctgcgagagcattctgcgggtctttcctttctgtttcagaatcacacctgttctcacaagggataaatttgtcaccttcagtttttatttcaggaacttccaataggtcttttttatgatctgttaaaacatactttgggactctaggtggtttggtttcttctgagaagttggagccactgtcccagccattttctgcactttcagagttactttcattgtcatcagaggagcagaagggtggctgagaatcatcaatcttgtctcttccatcatcagaatgaatcagaaagcactcgtctgcttcatcgctctctgcttttaaagactggatgccactgtcatttaaattttcacttacagtctgaacagatacatttttttcaaatttccccaagtgcattaaagacttgaccatgagctcttgataacaagagtatctgtcttccttcctactggagttttcttgtgcagttgaaagaagactttcatccataggttttatcatgatttcctctgcggtagagtgaccatgtgtttccaaggggccatcgtcctctgtcctgtcactgcggtcttcttggcagtctgcttttgggctgtagtgtcggggcttcattagcagggatttccttttgttgactggaacccccaaagcctgatcttcagctgttctcttctttgccatggagcaatcataggcaacactttttttctctgaatgacttggttcctttaaaggactctggtgtccctcaccaggtaagtggcctcatgtccacgggcacactgattctgagctcctggattagtgaatccattggcacctcggttcctttagagcgagtacgcagcgttttatcttcagcctctgcatccatcttccctaaaagctactggatctgaactggagagtttccatcactcctttacctggcgaacgtctacaggtgtgtcgaaagttatcttttcctggatgtgttccaaaatgctcttatgctatttctcttaggatttctccacgctgccccattcagaaattttattattttcttccacaactctgccaggcactggtttttgcgtgggatgatgccagcttctctcttcatgtggccttattaaaagccatggtttccgagatgtaaaacacccacagttacctcaattatttttctctccttacctctagtattcccctgaggtcacattcagttaaaaacatcctgcccttctccctacaaaaaggttccatagaatc

SEQ ID NO: 18710 - RNA, 4914 nt, Homo sapiens
  source 1..4914: mol_type = other RNA
tgagtgtgtgtgtgtgagtgtgtgtgtatattttgtagcatttgaagttttgtggcaagatttctatcaaattgaatgttgtcttgtttcctatggtgggtgagacccaaggtgccagtgtttgaagtaatcattcagattggagtagcattttttcatgtgttactatattttccattcctttccagtcaacccagtaagataaatgctatttcaggggatatggtatctacaaaatttttcatttggatgtgtttgtatttgctaagtacaaatctacaccaatattgtcacttgtatattgtaccaacatatggcaggaaagcctggctggtcacaccaagtcttatttttcatcttgggatacgagttgccaacgatctgatatgacttgaaaaacaaacagacaaatctgcatcactaaaaaggcttatgtttctttaaaacatttcaaataaataattcatattaacgaaaaccgtccagccaagtcgaatactttgctgattgctatatttaattattgctaacaaattctgagcaggctgttttccagcatcctgtgcttttgtgagtgcggattccccactagtgggcgccatttgtcttcttattccttccgtgcagctcaccttaccgcaaattcatttataaatacaaaaatcagtgaaaggtgggggaagaagtgtgcaataaaaatcaaactcaactatagtgcagtccttagacaaggatttccttcaccctttcctgtttcctcattaaaacccagcaagaaagatgacttgagaatagcatttctatttaaatcctattggaaaataaattaataaacacacttgtaaaaatacggcagacttcaaaatgcagttaaaagataaaaaactctttgattagtaataaataaattataaaaatgtcacatttattttacatatactttacaaaaaaaaaaagagtacaatgaagaaataaaagaaaaacatatgaaaataaataagatctaataattgactgcattgcttttaatccaagaagtctatcatagtttttctttcctttttatatcagctggggaaaataaaattagtgcaatgttgcaaattgtaaatgcagtacggcaacctccacgccttagcagtacatgaacctctaacagatccatctggagtttactgctgttggtaacttctgttgcccggcagcgctgtgatcctacacatggatacccttcactgcctgtttgatactttccagtagagctttgcattccggggaatagtcccgttccagattgctgtacatatctgtgagtgtatttacatatgcttcaaaattctgctcactgataggtcccatctgtggaagctggatgtcagcaaggcttgaaatgagagcttggcttagacctgccagctctttcagcagactttcattgttctgttctatgagtttgttctcctcctctatcgtctttaagttgctctccatagatgtgatctgggtctgaagtttcatcatatctgcttcaattttaaggttggattcattcagttcctttatttcttcatccaaatgcctaatttcttcatcactctctattcccccagttgctttgagcttgatggtcatgagttcttcagaaaccttgccctttttgataacttgtgcattgagaggacatccagataagcttcggtgggtgacaaaaacattatttacatggcccagcccattgcagcctggcaagggacaatgtggtagctcttgtttgttcagtttccaggagagggaggctccattgagaggattctccttctgtctcttggcagccagaggacagccagaagctgtgcggtgtgatgtgtatttacctgatatgtgaccttggccatcacaccctatcacaggacatttcagttcagggtcttctttttcttccttggtaggggtcattttgacaccacctttccttgcacgagggcatccggacaagcttctgtgggaagcatagtttccagtcacgtgccccgagccatcgcagcctggggttggacacttaagctcctgagagttggcagccatgagggattttagagtcttatctgctaaaggacatccagaaacactgcgatgagatgcatagtttcctgtcacgtggccacttccatcacatcctggtgttggacaggtgattagttcctttttgagatctcttgcatgaagcttgggtttagggcttggtatagaggcctctccaggaaactttttttcctctaaattttctagagagctcactgggtctttctctttctcctcctctgtcttcccgtgagttttgctatagttgataggagtgtcccagccctcttggtcacaaagagcctgatagaatgctgcattgaccagaatgctgcttgttttgaatggggaagaggaaggagttggaatagaagtgttagaggaagttaggggtgcagacttgtccaggattcgattttttttcatgcttaagtccaatgtgccattttcatccacttctatttcggctcccttggcatgcagactctgtggcttgttggagaggatgtctgtggcttccctgcagcgggtggaaaggttcaggatggcagcagctgctgctatgtgggtgtcttcactacattgaccgtagctataagagctggcacggccagggctctgggtgtgggcgcctgcactaggcagtcgattaggaaatttcactggatttggaaaatgctttgattcaggaaatggtggtgtttttcgtccttgcactgtttgtatgagagggcgtttaccgaaaacttgggcatcaaaactggcataatcaaatggtacttttccaaacttctcttgttcttttgacactgtggctctgggagaggtgatggcttgtgacgggaaattgaattcaatttgcttcaccaaacttgtcctgtgggcctggtcaggacactgcccagtttggggagaatcaagctgatttttatcctgggacattgccaatttttcagctgcagcaattggacaaccagaaagactcctgtgggtgttgcggttgctgttcacatgaccccttcctgtgcatcccggcgtgggacacttgagcacattttcatgcatggcaagaatttccaggggaacccgcactttgtgggggcaccccgaaaggctgcggtggtgcgggtagagccctgtcacgtgtcccgtgccatcacatccagggatcgggcacttggtctccctcttttcaggccttggtgaatgtttattgttaaagatttgtcttccacccatgtcgataactttggtttgcctcctttcccctgctaggtgctccagcaggaacctatccagctctttgtaggtgttatggaaaacacaacctcgctcagcctgcagagcaattgcctgctccagcaaacttaaattccccttggccttttccaggtcactaccctcttccgtcattactgccaggctctcgctatcttcctcctcaacgtcagggaatgagggctgggcattgccatccaggggttctgcgagagcattctgcgggtctttcctttctgtttcagaatcacactttgggactctaggtggtttggtttcttctgagaagttggagccactgtcccagccattttctgcactttcagagttactttcattgtcatcagaggagcagaagggtggctgagaatcatcaatcttgtctcttccatcatcagaatgaatcagaaagcactcgtctgcttcatcgctctctgcttttaaagactggatgccactgtcatttaaattttcacttacagtctgaacagatacatttttttcaaatttccccaagtgcattaaagacttgaccatgagctcttgataacaagagtatctgtcttccttcctactggagttttcttgtgcagttgaaagaagactttcatccataggttttatcatgatttcctctgcggtagagtgaccatgtgtttccaaggggccatcgtcctctgtcctgtcactgcggtcttcttggcagtctgcttttgggctgtagtgtcggggcttcattagcagggatttccttttgttgactggaacccccaaagcctgatcttcagctgttctcttctttgccatggagcaatcataggcaacactgagctcctggattagtgaatccattggcacctcggttcctttagagcgagtacgcagcgttttatcttcagcctctgcatccatctataaacagatgtataaagtgatttcctagtacttgtacttgacgtcttttcttactggagcttacatcaggggcaataagcaggtctcttccacatcgccccagtgcacagatctggtaccttcttttaggctgaagaggaagtcctggaattgctctctttttctccaggtaacttgtatgtcaactcagtttgccctgctgtgtcagggggactaaataaatgactttgtcttatttagtgataaatcctgaaattcattctttcttgcagaaaatttctaccgtcctgccttctctaccctttgcagtatatcaaagtgctcagctttttaatcatagatttctgtgtttcttgtaggatttgaccagacattaaatagatgcttcttcaacttaagtcagcaactgtagttccttccctaaaagctactggatctgaactggagagtttccatcactccttagtcttgatatgagcacgcagacacataaaatggaattgtcacaatgcttcagggacactcacaaaattgggggctttttttgtttgtttccaaaacttatatttctctcctccctggtgggctgaacggaaacactaaagctgtttctttgaaaggtagttcccatgatatgac

SEQ ID NO: 18711 - RNA, 4835 nt, Homo sapiens
  source 1..4835: mol_type = other RNA
tgagtgtgtgtgtgtgagtgtgtgtgtatattttgtagcatttgaagttttgtggcaagatttctatcaaattgaatgttgtcttgtttcctatggtgggtgagacccaaggtgccagtgtttgaagtaatcattcagattggagtagcattttttcatgtgttactatattttccattcctttccagtcaacccagtaagataaatgctatttcaggggatatggtatctacaaaatttttcatttggatgtgtttgtatttgctaagtacaaatctacaccaatattgtcacttgtatattgtaccaacatatggcaggaaagcctggctggtcacaccaagtcttatttttcatcttgggatacgagttgccaacgatctgatatgacttgaaaaacaaacagacaaatctgcatcactaaaaaggcttatgtttctttaaaacatttcaaataaataattcatattaacgaaaaccgtccagccaagtcgaatactttgctgattgctatatttaattattgctaacaaattctgagcaggctgttttccagcatcctgtgcttttgtgagtgcggattccccactagtgggcgccatttgtcttcttattccttccgtgcagctcaccttaccgcaaattcatttataaatacaaaaatcagtgaaaggtgggggaagaagtgtgcaataaaaatcaaactcaactatagtgcagtccttagacaaggatttccttcaccctttcctgtttcctcattaaaacccagcaagaaagatgacttgagaatagcatttctatttaaatcctattggaaaataaattaataaacacacttgtaaaaatacggcagacttcaaaatgcagttaaaagataaaaaactctttgattagtaataaataaattataaaaatgtcacatttattttacatatactttacaaaaaaaaaaagagtacaatgaagaaataaaagaaaaacatatgaaaataaataagatctaataattgactgcattgcttttaatccaagaagtctatcatagtttttctttcctttttatatcagctggggaaaataaaattagtgcaatgttgcaaattgtaaatgcagtacggcaacctccacgccttagcagtacatgaacctctaacagatccatctggagtttactgctgttggtaacttctgttgcccggcagcgctgtgatcctacacatggatacccttcactgcctgtttgatactttccagtagagctttgcattccggggaatagtcccgttccagattgctgtacatatctgtgagtgtatttacatatgcttcaaaattctgctcactgataggtcccatctgtggaagctggatgtcagcaaggcttgaaatgagagcttggcttagacctgccagctctttcagcagactttcattgttctgttctatgagtttgttctcctcctctatcgtctttaagttgctctccatagatgtgatctgggtctgaagtttcatcatatctgcttcaattttaaggttggattcattcagttcctttatttcttcatccaaatgcctaatttcttcatcactctctattcccccagttgctttgagcttgatggtcatgagttcttcagaaaccttgccctttttgataacttgtgcattgagaggacatccagataagcttcggtgggtgacaaaaacattatttacatggcccagcccattgcagcctggcaagggacaatgtggtagctcttgtttgttcagtttccaggagagggaggctccattgagaggattctccttctgtctcttggcagccagaggacagccagaagctgtgcggtgtgatgtgtatttacctgatatgtgaccttggccatcacaccctatcacaggacatttcagttcagggtcttctttttcttccttggtaggggtcattttgacaccacctttccttgcacgagggcatccggacaagcttctgtgggaagcatagtttccagtcacgtgccccgagccatcgcagcctggggttggacacttaagctcctgagagttggcagccatgagggattttagagtcttatctgctaaaggacatccagaaacactgcgatgagatgcatagtttcctgtcacgtggccacttccatcacatcctggtgttggacaggtgattagttcctttttgagatctcttgcatgaagcttgggtttagggcttggtatagaggcctctccaggaaactttttttcctctaaattttctagagagctcactgggtctttctctttctcctcctctgtcttcccgtgagttttgctatagttgataggagtgtcccagccctcttggtcacaaagagcctgatagaatgctgcattgaccagaatgctgcttgttttgaatggggaagaggaaggagttggaatagaagtgttagaggaagttaggggtgcagacttgtccaggattcgattttttttcatgcttaagtccaatgtgccattttcatccacttctatttcggctcccttggcatgcagactctgtggcttgttggagaggatgtctgtggcttccctgcagcgggtggaaaggttcaggatggcagcagctgctgctatgtgggtgtcttcactacattgaccgtagctataagagctggcacggccagggctctgggtgtgggcgcctgcactaggcagtcgattaggaaatttcactggatttggaaaatgctttgattcaggaaatggtggtgtttttcgtccttgcactgtttgtatgagagggcgtttaccgaaaacttgggcatcaaaactggcataatcaaatggtacttttccaaacttctcttgttcttttgacactgtggctctgggagaggtgatggcttgtgacgggaaattgaattcaatttgcttcaccaaacttgtcctgtgggcctggtcaggacactgcccagtttggggagaatcaagctgatttttatcctgggacattgccaatttttcagctgcagcaattggacaaccagaaagactcctgtgggtgttgcggttgctgttcacatgaccccttcctgtgcatcccggcgtgggacacttgagcacattttcatgcatggcaagaatttccaggggaacccgcactttgtgggggcaccccgaaaggctgcggtggtgcgggtagagccctgtcacgtgtcccgtgccatcacatccagggatcgggcacttggtctccctcttttcaggccttggtgaatgtttattgttaaagatttgtcttccacccatgtcgataactttggtttgcctcctttcccctgctaggtgctccagcaggaacctatccagctctttgtaggtgttatggaaaacacaacctcgctcagcctgcagagcaattgcctgctccagcaaacttaaattccccttggccttttccaggtcactaccctcttccgtcattactgccaggctctcgctatcttcctcctcaacgtcagggaatgagggctgggcattgccatccaggggttctgcgagagcattctgcgggtctttcctttctgtttcagaatcacactttgggactctaggtggtttggtttcttctgagaagttggagccactgtcccagccattttctgcactttcagagttactttcattgtcatcagaggagcagaagggtggctgagaatcatcaatcttgtctcttccatcatcagaatgaatcagaaagcactcgtctgcttcatcgctctctgcttttaaagactggatgccactgtcatttaaattttcacttacagtctgaacagatacatttttttcaaatttccccaagtgcattaaagacttgaccatgagctcttgataacaagagtatctgtcttccttcctactggagttttcttgtgcagttgaaagaagactttcatccataggttttatcatgatttcctctgcggtagagtgaccatgtgtttccaaggggccatcgtcctctgtcctgtcactgcggtcttcttggcagtctgcttttgggctgtagtgtcggggcttcattagcagggatttccttttgttgactggaacccccaaagcctgatcttcagctgttctcttctttgccatggagcaatcataggcaacactgagctcctggattagtgaatccattggcacctcggttcctttagagcgagtacgcagcgttttatcttcagcctctgcatccatctataaacagatgtataaagtgatttcctagtacttgtacttgacgtcttttcttactggagcttacatcaggggcaataagcaggtctcttccacatcgccccagtgcacagatctggtaccttcttttaggctgaagaggaagtcctggaattgctctctttttctccaggtaacttgtatgtcaactcagtttgccctgctgtgtcagggggactaaataaatgactttgtcttatttagtgataaatcctgaaattcattctttcttgcagaaaatttctaccgtcctgccttctctaccctttgcagtatatcaaagtgctcagctttttaatcatagatttctgtgtttcttgtaggatttgaccagacattaaatagatgcttcttcaacttaagtcagcaactgtagttccttccctaaaagctactggatctgaactggagagtttccatcactcttttttgtttgtttccaaaacttatatttctctcctccctggtgggctgaacggaaacactaaagctgtttctttgaaaggtagttcccatgatatgac

SEQ ID NO: 18712 - RNA, 4859 nt, Homo sapiens
  source 1..4859: mol_type = other RNA
tgagtgtgtgtgtgtgagtgtgtgtgtatattttgtagcatttgaagttttgtggcaagatttctatcaaattgaatgttgtcttgtttcctatggtgggtgagacccaaggtgccagtgtttgaagtaatcattcagattggagtagcattttttcatgtgttactatattttccattcctttccagtcaacccagtaagataaatgctatttcaggggatatggtatctacaaaatttttcatttggatgtgtttgtatttgctaagtacaaatctacaccaatattgtcacttgtatattgtaccaacatatggcaggaaagcctggctggtcacaccaagtcttatttttcatcttgggatacgagttgccaacgatctgatatgacttgaaaaacaaacagacaaatctgcatcactaaaaaggcttatgtttctttaaaacatttcaaataaataattcatattaacgaaaaccgtccagccaagtcgaatactttgctgattgctatatttaattattgctaacaaattctgagcaggctgttttccagcatcctgtgcttttgtgagtgcggattccccactagtgggcgccatttgtcttcttattccttccgtgcagctcaccttaccgcaaattcatttataaatacaaaaatcagtgaaaggtgggggaagaagtgtgcaataaaaatcaaactcaactatagtgcagtccttagacaaggatttccttcaccctttcctgtttcctcattaaaacccagcaagaaagatgacttgagaatagcatttctatttaaatcctattggaaaataaattaataaacacacttgtaaaaatacggcagacttcaaaatgcagttaaaagataaaaaactctttgattagtaataaataaattataaaaatgtcacatttattttacatatactttacaaaaaaaaaaagagtacaatgaagaaataaaagaaaaacatatgaaaataaataagatctaataattgactgcattgcttttaatccaagaagtctatcatagtttttctttcctttttatatcagctggggaaaataaaattagtgcaatgttgcaaattgtaaatgcagtacggcaacctccacgccttagcagtacatgaacctctaacagatccatctggagtttactgctgttggtaacttctgttgcccggcagcgctgtgatcctacacatggatacccttcactgcctgtttgatactttccagtagagctttgcattccggggaatagtcccgttccagattgctgtacatatctgtgagtgtatttacatatgcttcaaaattctgctcactgataggtcccatctgtggaagctggatgtcagcaaggcttgaaatgagagcttggcttagacctgccagctctttcagcagactttcattgttctgttctatgagtttgttctcctcctctatcgtctttaagttgctctccatagatgtgatctgggtctgaagtttcatcatatctgcttcaattttaaggttggattcattcagttcctttatttcttcatccaaatgcctaatttcttcatcactctctattcccccagttgctttgagcttgatggtcatgagttcttcagaaaccttgccctttttgataacttgtgcattgagaggacatccagataagcttcggtgggtgacaaaaacattatttacatggcccagcccattgcagcctggcaagggacaatgtggtagctcttgtttgttcagtttccaggagagggaggctccattgagaggattctccttctgtctcttggcagccagaggacagccagaagctgtgcggtgtgatgtgtatttacctgatatgtgaccttggccatcacaccctatcacaggacatttcagttcagggtcttctttttcttccttggtaggggtcattttgacaccacctttccttgcacgagggcatccggacaagcttctgtgggaagcatagtttccagtcacgtgccccgagccatcgcagcctggggttggacacttaagctcctgagagttggcagccatgagggattttagagtcttatctgctaaaggacatccagaaacactgcgatgagatgcatagtttcctgtcacgtggccacttccatcacatcctggtgttggacaggtgattagttcctttttgagatctcttgcatgaagcttgggtttagggcttggtatagaggcctctccaggaaactttttttcctctaaattttctagagagctcactgggtctttctctttctcctcctctgtcttcccgtgagttttgctatagttgataggagtgtcccagccctcttggtcacaaagagcctgatagaatgctgcattgaccagaatgctgcttgttttgaatggggaagaggaaggagttggaatagaagtgttagaggaagttaggggtgcagacttgtccaggattcgattttttttcatgcttaagtccaatgtgccattttcatccacttctatttcggctcccttggcatgcagactctgtggcttgttggagaggatgtctgtggcttccctgcagcgggtggaaaggttcaggatggcagcagctgctgctatgtgggtgtcttcactacattgaccgtagctataagagctggcacggccagggctctgggtgtgggcgcctgcactaggcagtcgattaggaaatttcactggatttggaaaatgctttgattcaggaaatggtggtgtttttcgtccttgcactgtttgtatgagagggcgtttaccgaaaacttgggcatcaaaactggcataatcaaatggtacttttccaaacttctcttgttcttttgacactgtggctctgggagaggtgatggcttgtgacgggaaattgaattcaatttgcttcaccaaacttgtcctgtgggcctggtcaggacactgcccagtttggggagaatcaagctgatttttatcctgggacattgccaatttttcagctgcagcaattggacaaccagaaagactcctgtgggtgttgcggttgctgttcacatgaccccttcctgtgcatcccggcgtgggacacttgagcacattttcatgcatggcaagaatttccaggggaacccgcactttgtgggggcaccccgaaaggctgcggtggtgcgggtagagccctgtcacgtgtcccgtgccatcacatccagggatcgggcacttggtctccctcttttcaggccttggtgaatgtttattgttaaagatttgtcttccacccatgtcgataactttggtttgcctcctttcccctgctaggtgctccagcaggaacctatccagctctttgtaggtgttatggaaaacacaacctcgctcagcctgcagagcaattgcctgctccagcaaacttaaattccccttggccttttccaggtcactaccctcttccgtcattactgccaggctctcgctatcttcctcctcaacgtcagggaatgagggctgggcattgccatccaggggttctgcgagagcattctgcgggtctttcctttctgtttcagaatcacactttgggactctaggtggtttggtttcttctgagaagttggagccactgtcccagccattttctgcactttcagagttactttcattgtcatcagaggagcagaagggtggctgagaatcatcaatcttgtctcttccatcatcagaatgaatcagaaagcactcgtctgcttcatcgctctctgcttttaaagactggatgccactgtcatttaaattttcacttacagtctgaacagatacatttttttcaaatttccccaagtgcattaaagacttgaccatgagctcttgataacaagagtatctgtcttccttcctactggagttttcttgtgcagttgaaagaagactttcatccataggttttatcatgatttcctctgcggtagagtgaccatgtgtttccaaggggccatcgtcctctgtcctgtcactgcggtcttcttggcagtctgcttttgggctgtagtgtcggggcttcattagcagggatttccttttgttgactggaacccccaaagcctgatcttcagctgttctcttctttgccatggagcaatcataggcaacactgagctcctggattagtgaatccattggcacctcggttcctttagagcgagtacgcagcgttttatcttcagcctctgcatccatctctctttttctccaggtaacttgtatgtcaactcagtttgccctgctgtgtcagggggactaaataaatgactttgtcttatttagtgataaatcctgaaattcattctttcttgcagaaaatttctaccgtcctgccttctctaccctttgcagtatatcaaagtgctcagctttttaatcatagatttctgtgtttcttgtaggatttgaccagacattaaatagatgcttcttcaacttaagtcagcaactgtagttccttccctaaaagctactggatctgaactggagagtttccatcactccttagtcttgatatgagcacgcagacacataaaatggaattgtcacaatgcttcagggacactcacaaaattgggggctctttacctggcgaacgtctacaggtgtgtcgaaagttatcttttcctggatgtgttccaaaatgctcttatgctatttctcttaggatttctccacgctgccccattcagaaattttattattttctctagtattcccctgaggtcacattcagttaaaaacatcctgcccttctccctacaaaaaggttccatagaatc

SEQ ID NO: 18713 - RNA, 3985 nt, Homo sapiens
  source 1..3985: mol_type = other RNA
tgagtgtgtgtgtgtgagtgtgtgtgtatattttgtagcatttgaagttttgtggcaagatttctatcaaattgaatgttgtcttgtttcctatggtgggtgagacccaaggtgccagtgtttgaagtaatcattcagattggagtagcattttttcatgtgttactatattttccattcctttccagtcaacccagtaagataaatgctatttcaggggatatggtatctacaaaatttttcatttggatgtgtttgtatttgctaagtacaaatctacaccaatattgtcacttgtatattgtaccaacatatggcaggaaagcctggctggtcacaccaagtcttatttttcatcttgggatacgagttgccaacgatctgatatgacttgaaaaacaaacagacaaatctgcatcactaaaaaggcttatgtttctttaaaacatttcaaataaataattcatattaacgaaaaccgtccagccaagtcgaatactttgctgattgctatatttaattattgctaacaaattctgagcaggctgttttccagcatcctgtgcttttgtgagtgcggattccccactagtgggcgccatttgtcttcttattccttccgtgcagctcaccttaccgcaaattcatttataaatacaaaaatcagtgaaaggtgggggaagaagtgtgcaataaaaatcaaactcaactatagtgcagtccttagacaaggatttccttcaccctttcctgtttcctcattaaaacccagcaagaaagatgacttgagaatagcatttctatttaaatcctattggaaaataaattaataaacacacttgtaaaaatacggcagacttcaaaatgcagttaaaagataaaaaactctttgattagtaataaataaattataaaaatgtcacatttattttacatatactttacaaaaaaaaaaagagtacaatgaagaaataaaagaaaaacatatgaaaataaataagatctaataattgactgcattgcttttaatccaagaagtctatcatagtttttctttcctttttatatcagctggggaaaataaaattagtgcaatgttgcaaattgtaaatgcagtacggcaacctccacgccttagcagtacatgaacctctaacagatccatctggagtttactgctgttggtaacttctgttgcccggcagcgctgtgatcctacacatggatacccttcactgcctgtttgatactttccagtagagctttgcattccggggaatagtcccgttccagattgctgtacatatctgtgagtgtatttacatatgcttcaaaattctgctcactgataggtcccatctgtggaagctggatgtcagcaaggcttgaaatgagagcttggcttagacctgccagctctttcagcagactttcattgttctgttctatgagtttgttctcctcctctatcgtctttaagttgctctccatagatgtgatctgggtctgaagtttcatcatatctgcttcaattttaaggttggattcattcagttcctttatttcttcatccaaatgcctaatttcttcatcactctctattcccccagttgctttgagcttgatggtcatgagttcttcagaaaccttgccctttttgataacttgtgcattgagaggacatccagataagcttcggtgggtgacaaaaacattatttacatggcccagcccattgcagcctggcaagggacaatgtggtagctcttgtttgttcagtttccaggagagggaggctccattgagaggattctccttctgtctcttggcagccagaggacagccagaagctgtgcggtgtgatgtgtatttacctgatatgtgaccttggccatcacaccctatcacaggacatttcagttcagggtcttctttttcttccttggtaggggtcattttgacaccacctttccttgcacgagggcatccggacaagcttctgtgggaagcatagtttccagtcacgtgccccgagccatcgcagcctggggttggacacttaagctcctgagagttggcagccatgagggattttagagtcttatctgctaaaggacatccagaaacactgcgatgagatgcatagtttcctgtcacgtggccacttccatcacatcctggtgttggacaggtgattagttcctttttgagatctcttgcatgaagcttgggtttagggcttggtatagaggcctctccaggaaactttttttcctctaaattttctagagagctcactgggtctttcttggcatgcagactctgtggcttgttggagaggatgtctgtggcttccctgcagcgggtggaaaggttcaggatggcagcagctgctgctatgtgggtgtcttcactacattgaccgtagctataagagctggcacggccagggctctgggtgtgggcgcctgcactaggcagtcgattaggaaatttcactggatttggaaaatgctttgattcaggaaatggtggtgtttttcgtccttgcactgtttgtatgagagggcgtttaccgaaaacttgggcatcaaaactggcataatcaaatggtacttttccaaacttctcttgttcttttgacactgtggctctgggagaggtgatggcttgtgacgggaaattgaattcaatttgcttcaccaaacttgtcctgtgggcctggtcaggacactgcccagtttggggagaatcaagctgatttttatcctgggacattgccaatttttcagctgcagcaattggacaaccagaaagactcctgtgggtgttgcggttgctgttcacatgaccccttcctgtgcatcccggcgtgggacacttgagcacattttcatgcatggcaagaatttccaggggaacccgcactttgtgggggcaccccgaaaggctgcggtggtgcgggtagagccctgtcacgtgtcccgtgccatcacatccagggatcgggcacttggtctccctcttttcaggccttggtgaatctgcggtagagtgaccatgtgtttccaaggggccatcgtcctctgtcctgtcactgcggtcttcttggcagtctgcttttgggctgtagtgtcggggcttcattagcagggatttccttttgttgactggaacccccaaagcctgatcttcagctgttctcttctttgccatggagcaatcataggcaacactgagctcctggattagtgaatccattggcacctcggttcctttagagcgagtacgcagcgttttatcttcagcctctgcatccatctataaacagatgtataaagtgatttcctagtacttgtacttgacgtcttttcttactggagcttacatcaggggcaataagcaggtctcttccacatcgccccagtgcacagatctggtaccttcttttaggctgaagaggaagtcctggaattgctctctttttctccaggtaacttgtatgtcaactcagtttgccctgctgtgtcagggggactaaataaatgactttgtcttatttagtgataaatcctgaaattcattctttcttgcagaaaatttctaccgtcctgccttctctaccctttgcagtatatcaaagtgctcagctttttaatcatagatttctgtgtttcttgtaggatttgaccagacattaaatagatgcttcttcaacttaagtcagcaactgtagttccttccctaaaagctactggatctgaactggagagtttccatcactcctttacctggcgaacgtctacaggtgtgtcgaaagttatcttttcctggatgtgttccaaaatgctcttatgctatttctcttaggatttctccacgctgccccattcagaaattttattattttctctagtattcccctgaggtcacattcagttaaaaacatcctgcccttctccctacaaaaaggttccatagaatc

SEQ ID NO: 18714 - RNA, 4759 nt, Homo sapiens
  source 1..4759: mol_type = other RNA
tgagtgtgtgtgtgtgagtgtgtgtgtatattttgtagcatttgaagttttgtggcaagatttctatcaaattgaatgttgtcttgtttcctatggtgggtgagacccaaggtgccagtgtttgaagtaatcattcagattggagtagcattttttcatgtgttactatattttccattcctttccagtcaacccagtaagataaatgctatttcaggggatatggtatctacaaaatttttcatttggatgtgtttgtatttgctaagtacaaatctacaccaatattgtcacttgtatattgtaccaacatatggcaggaaagcctggctggtcacaccaagtcttatttttcatcttgggatacgagttgccaacgatctgatatgacttgaaaaacaaacagacaaatctgcatcactaaaaaggcttatgtttctttaaaacatttcaaataaataattcatattaacgaaaaccgtccagccaagtcgaatactttgctgattgctatatttaattattgctaacaaattctgagcaggctgttttccagcatcctgtgcttttgtgagtgcggattccccactagtgggcgccatttgtcttcttattccttccgtgcagctcaccttaccgcaaattcatttataaatacaaaaatcagtgaaaggtgggggaagaagtgtgcaataaaaatcaaactcaactatagtgcagtccttagacaaggatttccttcaccctttcctgtttcctcattaaaacccagcaagaaagatgacttgagaatagcatttctatttaaatcctattggaaaataaattaataaacacacttgtaaaaatacggcagacttcaaaatgcagttaaaagataaaaaactctttgattagtaataaataaattataaaaatgtcacatttattttacatatactttacaaaaaaaaaaagagtacaatgaagaaataaaagaaaaacatatgaaaataaataagatctaataattgactgcattgcttttaatccaagaagtctatcatagtttttctttcctttttatatcagctggggaaaataaaattagtgcaatgttgcaaattgtaaatgcagtacggcaacctccacgccttagcagtacatgaacctctaacagatccatctggagtttactgctgttggtaacttctgttgcccggcagcgctgtgatcctacacatggatacccttcactgcctgtttgatactttccagtagagctttgcattccggggaatagtcccgttccagattgctgtacatatctgtgagtgtatttacatatgcttcaaaattctgctcactgataggtcccatctgtggaagctggatgtcagcaaggcttgaaatgagagcttggcttagacctgccagctctttcagcagactttcattgttctgttctatgagtttgttctcctcctctatcgtctttaagttgctctccatagatgtgatctgggtctgaagtttcatcatatctgcttcaattttaaggttggattcattcagttcctttatttcttcatccaaatgcctaatttcttcatcactctctattcccccagttgctttgagcttgatggtcatgagttcttcagaaaccttgccctttttgataacttgtgcattgagaggacatccagataagcttcggtgggtgacaaaaacattatttacatggcccagcccattgcagcctggcaagggacaatgtggtagctcttgtttgttcagtttccaggagagggaggctccattgagaggattctccttctgtctcttggcagccagaggacagccagaagctgtgcggtgtgatgtgtatttacctgatatgtgaccttggccatcacaccctatcacaggacatttcagttcagggtcttctttttcttccttggtaggggtcattttgacaccacctttccttgcacgagggcatccggacaagcttctgtgggaagcatagtttccagtcacgtgccccgagccatcgcagcctggggttggacacttaagctcctgagagttggcagccatgagggattttagagtcttatctgctaaaggacatccagaaacactgcgatgagatgcatagtttcctgtcacgtggccacttccatcacatcctggtgttggacaggtgattagttcctttttgagatctcttgcatgaagcttgggtttagggcttggtatagaggcctctccaggaaactttttttcctctaaattttctagagagctcactgggtctttcttggcatgcagactctgtggcttgttggagaggatgtctgtggcttccctgcagcgggtggaaaggttcaggatggcagcagctgctgctatgtgggtgtcttcactacattgaccgtagctataagagctggcacggccagggctctgggtgtgggcgcctgcactaggcagtcgattaggaaatttcactggatttggaaaatgctttgattcaggaaatggtggtgtttttcgtccttgcactgtttgtatgagagggcgtttaccgaaaacttgggcatcaaaactggcataatcaaatggtacttttccaaacttctcttgttcttttgacactgtggctctgggagaggtgatggcttgtgacgggaaattgaattcaatttgcttcaccaaacttgtcctgtgggcctggtcaggacactgcccagtttggggagaatcaagctgatttttatcctgggacattgccaatttttcagctgcagcaattggacaaccagaaagactcctgtgggtgttgcggttgctgttcacatgaccccttcctgtgcatcccggcgtgggacacttgagcacattttcatgcatggcaagaatttccaggggaacccgcactttgtgggggcaccccgaaaggctgcggtggtgcgggtagagccctgtcacgtgtcccgtgccatcacatccagggatcgggcacttggtctccctcttttcaggccttggtgaatgtttattgttaaagatttgtcttccacccatgtcgataactttggtttgcctcctttcccctgctaggtgctccagcaggaacctatccagctctttgtaggtgttatggaaaacacaacctcgctcagcctgcagagcaattgcctgctccagcaaacttaaattccccttggccttttccaggtcactaccctcttccgtcattactgccaggctctcgctatcttcctcctcaacgtcagggaatgagggctgggcattgccatccaggggttctgcgagagcattctgcgggtctttcctttctgtttcagaatcacacctgttctcacaagggataaatttgtcaccttcagtttttatttcaggaacttccaataggtcttttttatgatctgttaaaacatactttgggactctaggtggtttggtttcttctgagaagttggagccactgtcccagccattttctgcactttcagagttactttcattgtcatcagaggagcagaagggtggctgagaatcatcaatcttgtctcttccatcatcagaatgaatcagaaagcactcgtctgcttcatcgctctctgcttttaaagactggatgccactgtcatttaaattttcacttacagtctgaacagatacatttttttcaaatttccccaagtgcattaaagacttgaccatgagctcttgataacaagagtatctgtcttccttcctactggagttttcttgtgcagttgaaagaagactttcatccataggttttatcatgatttcctctgcggtagagtgaccatgtgtttccaaggggccatcgtcctctgtcctgtcactgcggtcttcttggcagtctgcttttgggctgtagtgtcggggcttcattagcagggatttccttttgttgactggaacccccaaagcctgatcttcagctgttctcttctttgccatggagcaatcataggcaacactgagctcctggattagtgaatccattggcacctcggttcctttagagcgagtacgcagcgttttatcttcagcctctgcatccataaacctataaacagatgtataaagtgatttcctagtacttgtacttgacgtcttttcttactggagcttacatcaggggcaataagcaggtctcttccacatcgccccagtgcacagatctggtaccttcttttaggctgaagaggaagtcctggaattgctctctttttctccaggtaacttgtatgtcaactcagtttgccctgctgtgtcagggggactaaataaatgactttgtcttatttagtgataaatcctgaaattcattctttcttgcagaaaatttctaccgtcctgccttctctaccctttgcagtatatcaaagtgctcagctttttaatcatagatttctgtgtttcttgtaggatttgaccagacattaaatagatgcttcttcaacttaagtcagcaactgtagttccttccctaaaagctactggatctgaactggagagtttccatcactccttagtcttgatatgagcacgcagacacataaaatggaattgtcacaatgcttcagggacactcacaaaattgggggctttttttgtttgtttccaaaacttatatttctctcctccctggtgggctgaacggaaacactaaagctgtttctttgaaaggtagttcccatgatatgac

SEQ ID NO: 18715 - RNA, 4781 nt, Homo sapiens
  source 1..4781: mol_type = other RNA
tgagtgtgtgtgtgtgagtgtgtgtgtatattttgtagcatttgaagttttgtggcaagatttctatcaaattgaatgttgtcttgtttcctatggtgggtgagacccaaggtgccagtgtttgaagtaatcattcagattggagtagcattttttcatgtgttactatattttccattcctttccagtcaacccagtaagataaatgctatttcaggggatatggtatctacaaaatttttcatttggatgtgtttgtatttgctaagtacaaatctacaccaatattgtcacttgtatattgtaccaacatatggcaggaaagcctggctggtcacaccaagtcttatttttcatcttgggatacgagttgccaacgatctgatatgacttgaaaaacaaacagacaaatctgcatcactaaaaaggcttatgtttctttaaaacatttcaaataaataattcatattaacgaaaaccgtccagccaagtcgaatactttgctgattgctatatttaattattgctaacaaattctgagcaggctgttttccagcatcctgtgcttttgtgagtgcggattccccactagtgggcgccatttgtcttcttattccttccgtgcagctcaccttaccgcaaattcatttataaatacaaaaatcagtgaaaggtgggggaagaagtgtgcaataaaaatcaaactcaactatagtgcagtccttagacaaggatttccttcaccctttcctgtttcctcattaaaacccagcaagaaagatgacttgagaatagcatttctatttaaatcctattggaaaataaattaataaacacacttgtaaaaatacggcagacttcaaaatgcagttaaaagataaaaaactctttgattagtaataaataaattataaaaatgtcacatttattttacatatactttacaaaaaaaaaaagagtacaatgaagaaataaaagaaaaacatatgaaaataaataagatctaataattgactgcattgcttttaatccaagaagtctatcatagtttttctttcctttttatatcagctggggaaaataaaattagtgcaatgttgcaaattgtaaatgcagtacggcaacctccacgccttagcagtacatgaacctctaacagatccatctggagtttactgctgttggtaacttctgttgcccggcagcgctgtgatcctacacatggatacccttcactgcctgtttgatactttccagtagagctttgcattccggggaatagtcccgttccagattgctgtacatatctgtgagtgtatttacatatgcttcaaaattctgctcactgataggtcccatctgtggaagctggatgtcagcaaggcttgaaatgagagcttggcttagacctgccagctctttcagcagactttcattgttctgttctatgagtttgttctcctcctctatcgtctttaagttgctctccatagatgtgatctgggtctgaagtttcatcatatctgcttcaattttaaggttggattcattcagttcctttatttcttcatccaaatgcctaatttcttcatcactctctattcccccagttgctttgagcttgatggtcatgagttcttcagaaaccttgccctttttgataacttgtgcattgagaggacatccagataagcttcggtgggtgacaaaaacattatttacatggcccagcccattgcagcctggcaagggacaatgtggtagctcttgtttgttcagtttccaggagagggaggctccattgagaggattctccttctgtctcttggcagccagaggacagccagaagctgtgcggtgtgatgtgtatttacctgatatgtgaccttggccatcacaccctatcacaggacatttcagttcagggtcttctttttcttccttggtaggggtcattttgacaccacctttccttgcacgagggcatccggacaagcttctgtgggaagcatagtttccagtcacgtgccccgagccatcgcagcctggggttggacacttaagctcctgagagttggcagccatgagggattttagagtcttatctgctaaaggacatccagaaacactgcgatgagatgcatagtttcctgtcacgtggccacttccatcacatcctggtgttggacaggtgattagttcctttttgagatctcttgcatgaagcttgggtttagggcttggtatagaggcctctccaggaaactttttttcctctaaattttctagagagctcactgggtctttcttggcatgcagactctgtggcttgttggagaggatgtctgtggcttccctgcagcgggtggaaaggttcaggatggcagcagctgctgctatgtgggtgtcttcactacattgaccgtagctataagagctggcacggccagggctctgggtgtgggcgcctgcactaggcagtcgattaggaaatttcactggatttggaaaatgctttgattcaggaaatggtggtgtttttcgtccttgcactgtttgtatgagagggcgtttaccgaaaacttgggcatcaaaactggcataatcaaatggtacttttccaaacttctcttgttcttttgacactgtggctctgggagaggtgatggcttgtgacgggaaattgaattcaatttgcttcaccaaacttgtcctgtgggcctggtcaggacactgcccagtttggggagaatcaagctgatttttatcctgggacattgccaatttttcagctgcagcaattggacaaccagaaagactcctgtgggtgttgcggttgctgttcacatgaccccttcctgtgcatcccggcgtgggacacttgagcacattttcatgcatggcaagaatttccaggggaacccgcactttgtgggggcaccccgaaaggctgcggtggtgcgggtagagccctgtcacgtgtcccgtgccatcacatccagggatcgggcacttggtctccctcttttcaggccttggtgaatgtttattgttaaagatttgtcttccacccatgtcgataactttggtttgcctcctttcccctgctaggtgctccagcaggaacctatccagctctttgtaggtgttatggaaaacacaacctcgctcagcctgcagagcaattgcctgctccagcaaacttaaattccccttggccttttccaggtcactaccctcttccgtcattactgccaggctctcgctatcttcctcctcaacgtcagggaatgagggctgggcattgccatccaggggttctgcgagagcattctgcgggtctttcctttctgtttcagaatcacacctgttctcacaagggataaatttgtcaccttcagtttttatttcaggaacttccaataggtcttttttatgatctgttaaaacatactttgggactctaggtggtttggtttcttctgagaagttggagccactgtcccagccattttctgcactttcagagttactttcattgtcatcagaggagcagaagggtggctgagaatcatcaatcttgtctcttccatcatcagaatgaatcagaaagcactcgtctgcttcatcgctctctgcttttaaagactggatgccactgtcatttaaattttcacttacagtctgaacagatacatttttttcaaatttccccaagtgcattaaagacttgaccatgagctcttgataacaagagtatctgtcttccttcctactggagttttcttgtgcagttgaaagaagactttcatccataggttttatcatgatttcctctgcggtagagtgaccatgtgtttccaaggggccatcgtcctctgtcctgtcactgcggtcttcttggcagtctgcttttgggctgtagtgtcggggcttcattagcagggatttccttttgttgactggaacccccaaagcctgatcttcagctgttctcttctttgccatggagcaatcataggcaacactgagctcctggattagtgaatccattggcacctcggttcctttagagcgagtacgcagcgttttatcttcagcctctgcatccataaacctataaacagatgtataaagtgatttcctagtacttgtacttgacgtcttttcttactggagcttacatcaggggcaataagcaggtctcttccacatcgccccagtgcacagatctggtaccttcttttaggctgaagaggaagtcctggaattgctctctttttctccaggtaacttgtatgtcaactcagtttgccctgctgtgtcagggggactaaataaatgactttgtcttatttagtgataaatcctgaaattcattctttcttgcagaaaatttctaccgtcctgccttctctaccctttgcagtatatcaaagtgctcagctttttaatcatagatttctgtgtttcttgtaggatttgaccagacattaaatagatgcttcttcaacttaagtcagcaactgtagttccttccctaaaagctactggatctgaactggagagtttccatcactcctttacctggcgaacgtctacaggtgtgtcgaaagttatcttttcctggatgtgttccaaaatgctcttatgctatttctcttaggatttctccacgctgccccattcagaaattttattattttctctagtattcccctgaggtcacattcagttaaaaacatcctgcccttctccctacaaaaaggttccatagaatc

SEQ ID NO: 18716 - RNA, 4856 nt, Homo sapiens
  source 1..4856: mol_type = other RNA
tgagtgtgtgtgtgtgagtgtgtgtgtatattttgtagcatttgaagttttgtggcaagatttctatcaaattgaatgttgtcttgtttcctatggtgggtgagacccaaggtgccagtgtttgaagtaatcattcagattggagtagcattttttcatgtgttactatattttccattcctttccagtcaacccagtaagataaatgctatttcaggggatatggtatctacaaaatttttcatttggatgtgtttgtatttgctaagtacaaatctacaccaatattgtcacttgtatattgtaccaacatatggcaggaaagcctggctggtcacaccaagtcttatttttcatcttgggatacgagttgccaacgatctgatatgacttgaaaaacaaacagacaaatctgcatcactaaaaaggcttatgtttctttaaaacatttcaaataaataattcatattaacgaaaaccgtccagccaagtcgaatactttgctgattgctatatttaattattgctaacaaattctgagcaggctgttttccagcatcctgtgcttttgtgagtgcggattccccactagtgggcgccatttgtcttcttattccttccgtgcagctcaccttaccgcaaattcatttataaatacaaaaatcagtgaaaggtgggggaagaagtgtgcaataaaaatcaaactcaactatagtgcagtccttagacaaggatttccttcaccctttcctgtttcctcattaaaacccagcaagaaagatgacttgagaatagcatttctatttaaatcctattggaaaataaattaataaacacacttgtaaaaatacggcagacttcaaaatgcagttaaaagataaaaaactctttgattagtaataaataaattataaaaatgtcacatttattttacatatactttacaaaaaaaaaaagagtacaatgaagaaataaaagaaaaacatatgaaaataaataagatctaataattgactgcattgcttttaatccaagaagtctatcatagtttttctttcctttttatatcagctggggaaaataaaattagtgcaatgttgcaaattgtaaatgcagtacggcaacctccacgccttagcagtacatgaacctctaacagatccatctggagtttactgctgttggtaacttctgttgcccggcagcgctgtgatcctacacatggatacccttcactgcctgtttgatactttccagtagagctttgcattccggggaatagtcccgttccagattgctgtacatatctgtgagtgtatttacatatgcttcaaaattctgctcactgataggtcccatctgtggaagctggatgtcagcaaggcttgaaatgagagcttggcttagacctgccagctctttcagcagactttcattgttctgttctatgagtttgttctcctcctctatcgtctttaagttgctctccatagatgtgatctgggtctgaagtttcatcatatctgcttcaattttaaggttggattcattcagttcctttatttcttcatccaaatgcctaatttcttcatcactctctattcccccagttgctttgagcttgatggtcatgagttcttcagaaaccttgccctttttgataacttgtgcattgagaggacatccagataagcttcggtgggtgacaaaaacattatttacatggcccagcccattgcagcctggcaagggacaatgtggtagctcttgtttgttcagtttccaggagagggaggctccattgagaggattctccttctgtctcttggcagccagaggacagccagaagctgtgcggtgtgatgtgtatttacctgatatgtgaccttggccatcacaccctatcacaggacatttcagttcagggtcttctttttcttccttggtaggggtcattttgacaccacctttccttgcacgagggcatccggacaagcttctgtgggaagcatagtttccagtcacgtgccccgagccatcgcagcctggggttggacacttaagctcctgagagttggcagccatgagggattttagagtcttatctgctaaaggacatccagaaacactgcgatgagatgcatagtttcctgtcacgtggccacttccatcacatcctggtgttggacaggtgattagttcctttttgagatctcttgcatgaagcttgggtttagggcttggtatagaggcctctccaggaaactttttttcctctaaattttctagagagctcactgggtctttcttggcatgcagactctgtggcttgttggagaggatgtctgtggcttccctgcagcgggtggaaaggttcaggatggcagcagctgctgctatgtgggtgtcttcactacattgaccgtagctataagagctggcacggccagggctctgggtgtgggcgcctgcactaggcagtcgattaggaaatttcactggatttggaaaatgctttgattcaggaaatggtggtgtttttcgtccttgcactgtttgtatgagagggcgtttaccgaaaacttgggcatcaaaactggcataatcaaatggtacttttccaaacttctcttgttcttttgacactgtggctctgggagaggtgatggcttgtgacgggaaattgaattcaatttgcttcaccaaacttgtcctgtgggcctggtcaggacactgcccagtttggggagaatcaagctgatttttatcctgggacattgccaatttttcagctgcagcaattggacaaccagaaagactcctgtgggtgttgcggttgctgttcacatgaccccttcctgtgcatcccggcgtgggacacttgagcacattttcatgcatggcaagaatttccaggggaacccgcactttgtgggggcaccccgaaaggctgcggtggtgcgggtagagccctgtcacgtgtcccgtgccatcacatccagggatcgggcacttggtctccctcttttcaggccttggtgaatgtttattgttaaagatttgtcttccacccatgtcgataactttggtttgcctcctttcccctgctaggtgctccagcaggaacctatccagctctttgtaggtgttatggaaaacacaacctcgctcagcctgcagagcaattgcctgctccagcaaacttaaattccccttggccttttccaggtcactaccctcttccgtcattactgccaggctctcgctatcttcctcctcaacgtcagggaatgagggctgggcattgccatccaggggttctgcgagagcattctgcgggtctttcctttctgtttcagaatcacacctgttctcacaagggataaatttgtcaccttcagtttttatttcaggaacttccaataggtcttttttatgatctgttaaaacatactttgggactctaggtggtttggtttcttctgagaagttggagccactgtcccagccattttctgcactttcagagttactttcattgtcatcagaggagcagaagggtggctgagaatcatcaatcttgtctcttccatcatcagaatgaatcagaaagcactcgtctgcttcatcgctctctgcttttaaagactggatgccactgtcatttaaattttcacttacagtctgaacagatacatttttttcaaatttccccaagtgcattaaagacttgaccatgagctcttgataacaagagtatctgtcttccttcctactggagttttcttgtgcagttgaaagaagactttcatccataggttttatcatgatttcctctgcggtagagtgaccatgtgtttccaaggggccatcgtcctctgtcctgtcactgcggtcttcttggcagtctgcttttgggctgtagtgtcggggcttcattagcagggatttccttttgttgactggaacccccaaagcctgatcttcagctgttctcttctttgccatggagcaatcataggcaacactgagctcctggattagtgaatccattggcacctcggttcctttagagcgagtacgcagcgttttatcttcagcctctgcatccatctataaacagatgtataaagtgatttcctagtacttgtacttgacgtcttttcttactggagcttacatcaggggcaataagcaggtctcttccacatcgccccagtgcacagatctggtaccttcttttaggctgaagaggaagtcctggaattgctctctttttctccaggtaacttgtatgtcaactcagtttgccctgctgtgtcagggggactaaataaatgactttgtcttatttagtgataaatcctgaaattcattctttcttgcagaaaatttctaccgtcctgccttctctaccctttgcagtatatcaaagtgctcagctttttaatcatagatttctgtgtttcttgtaggatttgaccagacattaaatagatgcttcttcaacttaagtcagcaactgtagttccttccctaaaagctactggatctgaactggagagtttccatcactccttagtcttgatatgagcacgcagacacataaaatggaattgtcacaatgcttcagggacactcacaaaattgggggctctttacctggcgaacgtctacaggtgtgtcgaaagttatcttttcctggatgtgttccaaaatgctcttatgctatttctcttaggatttctccacgctgccccattcagaaattttattattttctctagtattcccctgaggtcacattcagttaaaaacatcctgcccttctccctacaaaaaggttccatagaatc

SEQ ID NO: 18717 - RNA, 4823 nt, Homo sapiens
  source 1..4823: mol_type = other RNA
tgagtgtgtgtgtgtgagtgtgtgtgtatattttgtagcatttgaagttttgtggcaagatttctatcaaattgaatgttgtcttgtttcctatggtgggtgagacccaaggtgccagtgtttgaagtaatcattcagattggagtagcattttttcatgtgttactatattttccattcctttccagtcaacccagtaagataaatgctatttcaggggatatggtatctacaaaatttttcatttggatgtgtttgtatttgctaagtacaaatctacaccaatattgtcacttgtatattgtaccaacatatggcaggaaagcctggctggtcacaccaagtcttatttttcatcttgggatacgagttgccaacgatctgatatgacttgaaaaacaaacagacaaatctgcatcactaaaaaggcttatgtttctttaaaacatttcaaataaataattcatattaacgaaaaccgtccagccaagtcgaatactttgctgattgctatatttaattattgctaacaaattctgagcaggctgttttccagcatcctgtgcttttgtgagtgcggattccccactagtgggcgccatttgtcttcttattccttccgtgcagctcaccttaccgcaaattcatttataaatacaaaaatcagtgaaaggtgggggaagaagtgtgcaataaaaatcaaactcaactatagtgcagtccttagacaaggatttccttcaccctttcctgtttcctcattaaaacccagcaagaaagatgacttgagaatagcatttctatttaaatcctattggaaaataaattaataaacacacttgtaaaaatacggcagacttcaaaatgcagttaaaagataaaaaactctttgattagtaataaataaattataaaaatgtcacatttattttacatatactttacaaaaaaaaaaagagtacaatgaagaaataaaagaaaaacatatgaaaataaataagatctaataattgactgcattgcttttaatccaagaagtctatcatagtttttctttcctttttatatcagctggggaaaataaaattagtgcaatgttgcaaattgtaaatgcagtacggcaacctccacgccttagcagtacatgaacctctaacagatccatctggagtttactgctgttggtaacttctgttgcccggcagcgctgtgatcctacacatggatacccttcactgcctgtttgatactttccagtagagctttgcattccggggaatagtcccgttccagattgctgtacatatctgtgagtgtatttacatatgcttcaaaattctgctcactgataggtcccatctgtggaagctggatgtcagcaaggcttgaaatgagagcttggcttagacctgccagctctttcagcagactttcattgttctgttctatgagtttgttctcctcctctatcgtctttaagttgctctccatagatgtgatctgggtctgaagtttcatcatatctgcttcaattttaaggttggattcattcagttcctttatttcttcatccaaatgcctaatttcttcatcactctctattcccccagttgctttgagcttgatggtcatgagttcttcagaaaccttgccctttttgataacttgtgcattgagaggacatccagataagcttcggtgggtgacaaaaacattatttacatggcccagcccattgcagcctggcaagggacaatgtggtagctcttgtttgttcagtttccaggagagggaggctccattgagaggattctccttctgtctcttggcagccagaggacagccagaagctgtgcggtgtgatgtgtatttacctgatatgtgaccttggccatcacaccctatcacaggacatttcagttcagggtcttctttttcttccttggtaggggtcattttgacaccacctttccttgcacgagggcatccggacaagcttctgtgggaagcatagtttccagtcacgtgccccgagccatcgcagcctggggttggacacttaagctcctgagagttggcagccatgagggattttagagtcttatctgctaaaggacatccagaaacactgcgatgagatgcatagtttcctgtcacgtggccacttccatcacatcctggtgttggacaggtgattagttcctttttgagatctcttgcatgaagcttgggtttagggcttggtatagaggcctctccaggaaactttttttcctctaaattttctagagagctcactgggtctttcttggcatgcagactctgtggcttgttggagaggatgtctgtggcttccctgcagcgggtggaaaggttcaggatggcagcagctgctgctatgtgggtgtcttcactacattgaccgtagctataagagctggcacggccagggctctgggtgtgggcgcctgcactaggcagtcgattaggaaatttcactggatttggaaaatgctttgattcaggaaatggtggtgtttttcgtccttgcactgtttgtatgagagggcgtttaccgaaaacttgggcatcaaaactggcataatcaaatggtacttttccaaacttctcttgttcttttgacactgtggctctgggagaggtgatggcttgtgacgggaaattgaattcaatttgcttcaccaaacttgtcctgtgggcctggtcaggacactgcccagtttggggagaatcaagctgatttttatcctgggacattgccaatttttcagctgcagcaattggacaaccagaaagactcctgtgggtgttgcggttgctgttcacatgaccccttcctgtgcatcccggcgtgggacacttgagcacattttcatgcatggcaagaatttccaggggaacccgcactttgtgggggcaccccgaaaggctgcggtggtgcgggtagagccctgtcacgtgtcccgtgccatcacatccagggatcgggcacttggtctccctcttttcaggccttggtgaatgtttattgttaaagatttgtcttccacccatgtcgataactttggtttgcctcctttcccctgctaggtgctccagcaggaacctatccagctctttgtaggtgttatggaaaacacaacctcgctcagcctgcagagcaattgcctgctccagcaaacttaaattccccttggccttttccaggtcactaccctcttccgtcattactgccaggctctcgctatcttcctcctcaacgtcagggaatgagggctgggcattgccatccaggggttctgcgagagcattctgcgggtctttcctttctgtttcagaatcacacctgttctcacaagggataaatttgtcaccttcagtttttatttcaggaacttccaataggtcttttttatgatctgttaaaacatactttgggactctaggtggtttggtttcttctgagaagttggagccactgtcccagccattttctgcactttcagagttactttcattgtcatcagaggagcagaagggtggctgagaatcatcaatcttgtctcttccatcatcagaatgaatcagaaagcactcgtctgcttcatcgctctctgcttttaaagactggatgccactgtcatttaaattttcacttacagtctgaacagatacatttttttcaaatttccccaagtgcattaaagacttgaccatgagctcttgataacaagagtatctgtcttccttcctactggagttttcttgtgcagttgaaagaagactttcatccataggttttatcatgatttcctctgcggtagagtgaccatgtgtttccaaggggccatcgtcctctgtcctgtcactgcggtcttcttggcagtctgcttttgggctgtagtgtcggggcttcattagcagggatttccttttgttgactggaacccccaaagcctgatcttcagctgttctcttctttgccatggagcaatcataggcaacactgagctcctggattagtgaatccattggcacctcggttcctttagagcgagtacgcagcgttttatcttcagcctctgcatccatctataacatgaacacaaagtcctgaggtcattcaaacctataaacagatgtataaagtgatttcctagtacttgtacttgacgtcttttcttactggagcttacatcaggggcaataagcaggtctcttccacatcgccccagtgcacagatctggtaccttcttttaggctgaagaggaagtcctggaattgctctctttttctccaggtaacttgtatgtcaactcagtttgccctgctgtgtcagggggactaaataaatgactttgtcttatttagtgataaatcctgaaattcattctttcttgcagaaaatttctaccgtcctgccttctctaccctttgcagtatatcaaagtgctcagctttttaatcatagatttctgtgtttcttgtaggatttgaccagacattaaatagatgcttcttcaacttaagtcagcaactgtagttccttccctaaaagctactggatctgaactggagagtttccatcactccttagtcttgatatgagcacgcagacacataaaatggaattgtcacaatgcttcagggacactcacaaaattgggggctcggtgcctcctagcctttgttctgcctctcacgctgacatcagggaagcagtgatgtagaataaagcaggggtgggctaggttagtccagtgtttgtgtcgttgtgtggtgtgcagggacactctgtgat

SEQ ID NO: 18718 - RNA, 4621 nt, Homo sapiens
  source 1..4621: mol_type = other RNA
tgagtgtgtgtgtgtgagtgtgtgtgtatattttgtagcatttgaagttttgtggcaagatttctatcaaattgaatgttgtcttgtttcctatggtgggtgagacccaaggtgccagtgtttgaagtaatcattcagattggagtagcattttttcatgtgttactatattttccattcctttccagtcaacccagtaagataaatgctatttcaggggatatggtatctacaaaatttttcatttggatgtgtttgtatttgctaagtacaaatctacaccaatattgtcacttgtatattgtaccaacatatggcaggaaagcctggctggtcacaccaagtcttatttttcatcttgggatacgagttgccaacgatctgatatgacttgaaaaacaaacagacaaatctgcatcactaaaaaggcttatgtttctttaaaacatttcaaataaataattcatattaacgaaaaccgtccagccaagtcgaatactttgctgattgctatatttaattattgctaacaaattctgagcaggctgttttccagcatcctgtgcttttgtgagtgcggattccccactagtgggcgccatttgtcttcttattccttccgtgcagctcaccttaccgcaaattcatttataaatacaaaaatcagtgaaaggtgggggaagaagtgtgcaataaaaatcaaactcaactatagtgcagtccttagacaaggatttccttcaccctttcctgtttcctcattaaaacccagcaagaaagatgacttgagaatagcatttctatttaaatcctattggaaaataaattaataaacacacttgtaaaaatacggcagacttcaaaatgcagttaaaagataaaaaactctttgattagtaataaataaattataaaaatgtcacatttattttacatatactttacaaaaaaaaaaagagtacaatgaagaaataaaagaaaaacatatgaaaataaataagatctaataattgactgcattgcttttaatccaagaagtctatcatagtttttctttcctttttatatcagctggggaaaataaaattagtgcaatgttgcaaattgtaaatgcagtacggcaacctccacgccttagcagtacatgaacctctaacagatccatctggagtttactgctgttggtaacttctgttgcccggcagcgctgtgatcctacacatggatacccttcactgcctgtttgatactttccagtagagctttgcattccggggaatagtcccgttccagattgctgtacatatctgtgagtgtatttacatatgcttcaaaattctgctcactgataggtcccatctgtggaagctggatgtcagcaaggcttgaaatgagagcttggcttagacctgccagctctttcagcagactttcattgttctgttctatgagtttgttctcctcctctatcgtctttaagttgctctccatagatgtgatctgggtctgaagtttcatcatatctgcttcaattttaaggttggattcattcagttcctttatttcttcatccaaatgcctaatttcttcatcactctctattcccccagttgctttgagcttgatggtcatgagttcttcagaaaccttgccctttttgataacttgtgcattgagaggacatccagataagcttcggtgggtgacaaaaacattatttacatggcccagcccattgcagcctggcaagggacaatgtggtagctcttgtttgttcagtttccaggagagggaggctccattgagaggattctccttctgtctcttggcagccagaggacagccagaagctgtgcggtgtgatgtgtatttacctgatatgtgaccttggccatcacaccctatcacaggacatttcagttcagggtcttctttttcttccttggtaggggtcattttgacaccacctttccttgcacgagggcatccggacaagcttctgtgggaagcatagtttccagtcacgtgccccgagccatcgcagcctggggttggacacttaagctcctgagagttggcagccatgagggattttagagtcttatctgctaaaggacatccagaaacactgcgatgagatgcatagtttcctgtcacgtggccacttccatcacatcctggtgttggacaggtgattagttcctttttgagatctcttgcatgaagcttgggtttagggcttggtatagaggcctctccaggaaactttttttcctctaaattttctagagagctcactgggtctttcttggcatgcagactctgtggcttgttggagaggatgtctgtggcttccctgcagcgggtggaaaggttcaggatggcagcagctgctgctatgtgggtgtcttcactacattgaccgtagctataagagctggcacggccagggctctgggtgtgggcgcctgcactaggcagtcgattaggaaatttcactggatttggaaaatgctttgattcaggaaatggtggtgtttttcgtccttgcactgtttgtatgagagggcgtttaccgaaaacttgggcatcaaaactggcataatcaaatggtacttttccaaacttctcttgttcttttgacactgtggctctgggagaggtgatggcttgtgacgggaaattgaattcaatttgcttcaccaaacttgtcctgtgggcctggtcaggacactgcccagtttggggagaatcaagctgatttttatcctgggacattgccaatttttcagctgcagcaattggacaaccagaaagactcctgtgggtgttgcggttgctgttcacatgaccccttcctgtgcatcccggcgtgggacacttgagcacattttcatgcatggcaagaatttccaggggaacccgcactttgtgggggcaccccgaaaggctgcggtggtgcgggtagagccctgtcacgtgtcccgtgccatcacatccagggatcgggcacttggtctccctcttttcaggccttggtgaatgtttattgttaaagatttgtcttccacccatgtcgataactttggtttgcctcctttcccctgctaggtgctccagcaggaacctatccagctctttgtaggtgttatggaaaacacaacctcgctcagcctgcagagcaattgcctgctccagcaaacttaaattccccttggccttttccaggtcactaccctcttccgtcattactgccaggctctcgctatcttcctcctcaacgtcagggaatgagggctgggcattgccatccaggggttctgcgagagcattctgcgggtctttcctttctgtttcagaatcacacctgttctcacaagggataaatttgtcaccttcagtttttatttcaggaacttccaataggtcttttttatgatctgttaaaacatactttgggactctaggtggtttggtttcttctgagaagttggagccactgtcccagccattttctgcactttcagagttactttcattgtcatcagaggagcagaagggtggctgagaatcatcaatcttgtctcttccatcatcagaatgaatcagaaagcactcgtctgcttcatcgctctctgcttttaaagactggatgccactgtcatttaaattttcacttacagtctgaacagatacatttttttcaaatttccccaagtgcattaaagacttgaccatgagctcttgataacaagagtatctgtcttccttcctactggagttttcttgtgcagttgaaagaagactttcatccataggttttatcatgatttcctctgcggtagagtgaccatgtgtttccaaggggccatcgtcctctgtcctgtcactgcggtcttcttggcagtctgcttttgggctgtagtgtcggggcttcattagcagggatttccttttgttgactggaacccccaaagcctgatcttcagctgttctcttctttgccatggagcaatcataggcaacactgagctcctggattagtgaatccattggcacctcggttcctttagagcgagtacgcagcgttttatcttcagcctctgcatccatctctctttttctccaggtaacttgtatgtcaactcagtttgccctgctgtgtcagggggactaaataaatgactttgtcttatttagtgataaatcctgaaattcattctttcttgcagaaaatttctaccgtcctgccttctctaccctttgcagtatatcaaagtgctcagctttttaatcatagatttctgtgtttcttgtaggatttgaccagacattaaatagatgcttcttcaacttaagtcagcaactgtagttccttccctaaaagctactggatctgaactggagagtttccatcactcctttacctggcgaacgtctacaggtgtgtcgaaagttatcttttcctggatgtgttccaaaatgctcttatgctatttctcttaggatttctccacgctgccccattcagaaattttattattttctctagtattcccctgaggtcacattcagttaaaaacatcctgcccttctccctacaaaaaggttccatagaatc

SEQ ID NO: 18719 - RNA, 4359 nt, Homo sapiens
  source 1..4359: mol_type = other RNA
tgagtgtgtgtgtgtgagtgtgtgtgtatattttgtagcatttgaagttttgtggcaagatttctatcaaattgaatgttgtcttgtttcctatggtgggtgagacccaaggtgccagtgtttgaagtaatcattcagattggagtagcattttttcatgtgttactatattttccattcctttccagtcaacccagtaagataaatgctatttcaggggatatggtatctacaaaatttttcatttggatgtgtttgtatttgctaagtacaaatctacaccaatattgtcacttgtatattgtaccaacatatggcaggaaagcctggctggtcacaccaagtcttatttttcatcttgggatacgagttgccaacgatctgatatgacttgaaaaacaaacagacaaatctgcatcactaaaaaggcttatgtttctttaaaacatttcaaataaataattcatattaacgaaaaccgtccagccaagtcgaatactttgctgattgctatatttaattattgctaacaaattctgagcaggctgttttccagcatcctgtgcttttgtgagtgcggattccccactagtgggcgccatttgtcttcttattccttccgtgcagctcaccttaccgcaaattcatttataaatacaaaaatcagtgaaaggtgggggaagaagtgtgcaataaaaatcaaactcaactatagtgcagtccttagacaaggatttccttcaccctttcctgtttcctcattaaaacccagcaagaaagatgacttgagaatagcatttctatttaaatcctattggaaaataaattaataaacacacttgtaaaaatacggcagacttcaaaatgcagttaaaagataaaaaactctttgattagtaataaataaattataaaaatgtcacatttattttacatatactttacaaaaaaaaaaagagtacaatgaagaaataaaagaaaaacatatgaaaataaataagatctaataattgactgcattgcttttaatccaagaagtctatcatagtttttctttcctttttatatcagctggggaaaataaaattagtgcaatgttgcaaattgtaaatgcagtacggcaacctccacgccttagcagtacatgaacctctaacagatccatctggagtttactgctgttggtaacttctgttgcccggcagcgctgtgatcctacacatggatacccttcactgcctgtttgatactttccagtagagctttgcattccggggaatagtcccgttccagattgctgtacatatctgtgagtgtatttacatatgcttcaaaattctgctcactgataggtcccatctgtggaagctggatgtcagcaaggcttgaaatgagagcttggcttagacctgccagctctttcagcagactttcattgttctgttctatgagtttgttctcctcctctatcgtctttaagttgctctccatagatgtgatctgggtctgaagtttcatcatatctgcttcaattttaaggttggattcattcagttcctttatttcttcatccaaatgcctaatttcttcatcactctctattcccccagttgctttgagcttgatggtcatgagttcttcagaaaccttgccctttttgataacttgtgcattgagaggacatccagataagcttcggtgggtgacaaaaacattatttacatggcccagcccattgcagcctggcaagggacaatgtggtagctcttgtttgttcagtttccaggagagggaggctccattgagaggattctccttctgtctcttggcagccagaggacagccagaagctgtgcggtgtgatgtgtatttacctgatatgtgaccttggccatcacaccctatcacaggacatttcagttcagggtcttctttttcttccttggtaggggtcattttgacaccacctttccttgcacgagggcatccggacaagcttctgtgggaagcatagtttccagtcacgtgccccgagccatcgcagcctggggttggacacttaagctcctgagagttggcagccatgagggattttagagtcttatctgctaaaggacatccagaaacactgcgatgagatgcatagtttcctgtcacgtggccacttccatcacatcctggtgttggacaggtgattagttcctttttgagatctcttgcatgaagcttgggtttagggcttggtatagaggcctctccaggaaactttttttcctctaaattttctagagagctcactgggtctttcttggcatgcagactctgtggcttgttggagaggatgtctgtggcttccctgcagcgggtggaaaggttcaggatggcagcagctgctgctatgtgggtgtcttcactacattgaccgtagctataagagctggcacggccagggctctgggtgtgggcgcctgcactaggcagtcgattaggaaatttcactggatttggaaaatgctttgattcaggaaatggtggtgtttttcgtccttgcactgtttgtatgagagggcgtttaccgaaaacttgggcatcaaaactggcataatcaaatggtacttttccaaacttctcttgttcttttgacactgtggctctgggagaggtgatggcttgtgacgggaaattgaattcaatttgcttcaccaaacttgtcctgtgggcctggtcaggacactgcccagtttggggagaatcaagctgatttttatcctgggacattgccaatttttcagctgcagcaattggacaaccagaaagactcctgtgggtgttgcggttgctgttcacatgaccccttcctgtgcatcccggcgtgggacacttgagcacattttcatgcatggcaagaatttccaggggaacccgcactttgtgggggcaccccgaaaggctgcggtggtgcgggtagagccctgtcacgtgtcccgtgccatcacatccagggatcgggcacttggtctccctcttttcaggccttggtgaatgtttattgttaaagatttgtcttccacccatgtcgataactttggtttgcctcctttcccctgctaggtgctccagcaggaacctatccagctctttgtaggtgttatggaaaacacaacctcgctcagcctgcagagcaattgcctgctccagcaaacttaaattccccttggccttttccaggtcactaccctcttccgtcattactgccaggctctcgctatcttcctcctcaacgtcagggaatgagggctgggcattgccatccaggggttctgcgagagcattctgcgggtctttcctttctgtttcagaatcacacctgttctcacaagggataaatttgtcaccttcagtttttatttcaggaacttccaataggtcttttttatgatctgttaaaacatactttgggactctaggtggtttggtttcttctgagaagttggagccactgtcccagccattttctgcactttcagagttactttcattgtcatcagaggagcagaagggtggctgagaatcatcaatcttgtctcttccatcatcagaatgaatcagaaagcactcgtctgcttcatcgctctctgcttttaaagactggatgccactgtcatttaaattttcacttacagtctgaacagatacatttttttcaaatttccccaagtgcattaaagacttgaccatgagctcttgataacaagagtatctgtcttccttcctactggagttttcttgtgcagttgaaagaagactttcatccataggttttatcatgatttcctctgcggtagagtgaccatgtgtttccaaggggccatcgtcctctgtcctgtcactgcggtcttcttggcagtctgcttttgggctgtagtgtcggggcttcattagcagggatttccttttgttgactggaacccccaaagcctgatcttcagctgttctcttctttgccatggagcaatcataggcaacactgagctcctggattagtgaatccattggcacctcggttcctttagagcgagtacgcagcgttttatcttcagcctctgcatccatcttccctaaaagctactggatctgaactggagagtttccatcactcctttacctggcgaacgtctacaggtgtgtcgaaagttatcttttcctggatgtgttccaaaatgctcttatgctatttctcttaggatttctccacgctgccccattcagaaattttattattttctctagtattcccctgaggtcacattcagttaaaaacatcctgcccttctccctacaaaaaggttccatagaatc

SEQ ID NO: 18720 - RNA, 4258 nt, Homo sapiens
  source 1..4258: mol_type = other RNA
tgagtgtgtgtgtgtgagtgtgtgtgtatattttgtagcatttgaagttttgtggcaagatttctatcaaattgaatgttgtcttgtttcctatggtgggtgagacccaaggtgccagtgtttgaagtaatcattcagattggagtagcattttttcatgtgttactatattttccattcctttccagtcaacccagtaagataaatgctatttcaggggatatggtatctacaaaatttttcatttggatgtgtttgtatttgctaagtacaaatctacaccaatattgtcacttgtatattgtaccaacatatggcaggaaagcctggctggtcacaccaagtcttatttttcatcttgggatacgagttgccaacgatctgatatgacttgaaaaacaaacagacaaatctgcatcactaaaaaggcttatgtttctttaaaacatttcaaataaataattcatattaacgaaaaccgtccagccaagtcgaatactttgctgattgctatatttaattattgctaacaaattctgagcaggctgttttccagcatcctgtgcttttgtgagtgcggattccccactagtgggcgccatttgtcttcttattccttccgtgcagctcaccttaccgcaaattcatttataaatacaaaaatcagtgaaaggtgggggaagaagtgtgcaataaaaatcaaactcaactatagtgcagtccttagacaaggatttccttcaccctttcctgtttcctcattaaaacccagcaagaaagatgacttgagaatagcatttctatttaaatcctattggaaaataaattaataaacacacttgtaaaaatacggcagacttcaaaatgcagttaaaagataaaaaactctttgattagtaataaataaattataaaaatgtcacatttattttacatatactttacaaaaaaaaaaagagtacaatgaagaaataaaagaaaaacatatgaaaataaataagatctaataattgactgcattgcttttaatccaagaagtctatcatagtttttctttcctttttatatcagctggggaaaataaaattagtgcaatgttgcaaattgtaaatgcagtacggcaacctccacgccttagcagtacatgaacctctaacagatccatctggagtttactgctgttggtaacttctgttgcccggcagcgctgtgatcctacacatggatacccttcactgcctgtttgatactttccagtagagctttgcattccggggaatagtcccgttccagattgctgtacatatctgtgagtgtatttacatatgcttcaaaattctgctcactgataggtcccatctgtggaagctggatgtcagcaaggcttgaaatgagagcttggcttagacctgccagctctttcagcagactttcattgttctgttctatgagtttgttctcctcctctatcgtctttaagttgctctccatagatgtgatctgggtctgaagtttcatcatatctgcttcaattttaaggttggattcattcagttcctttatttcttcatccaaatgcctaatttcttcatcactctctattcccccagttgctttgagcttgatggtcatgagttcttcagaaaccttgccctttttgataacttgtgcattgagaggacatccagataagcttcggtgggtgacaaaaacattatttacatggcccagcccattgcagcctggcaagggacaatgtggtagctcttgtttgttcagtttccaggagagggaggctccattgagaggattctccttctgtctcttggcagccagaggacagccagaagctgtgcggtgtgatgtgtatttacctgatatgtgaccttggccatcacaccctatcacaggacatttcagttcagggtcttctttttcttccttggtaggggtcattttgacaccacctttccttgcacgagggcatccggacaagcttctgtgggaagcatagtttccagtcacgtgccccgagccatcgcagcctggggttggacacttaagctcctgagagttggcagccatgagggattttagagtcttatctgctaaaggacatccagaaacactgcgatgagatgcatagtttcctgtcacgtggccacttccatcacatcctggtgttggacaggtgattagttcctttttgagatctcttgcatgaagcttgggtttagggcttggtatagaggcctctccaggaaactttttttcctctaaattttctagagagctcactgggtctttcttggcatgcagactctgtggcttgttggagaggatgtctgtggcttccctgcagcgggtggaaaggttcaggatggcagcagctgctgctatgtgggtgtcttcactacattgaccgtagctataagagctggcacggccagggctctgggtgtgggcgcctgcactaggcagtcgattaggaaatttcactggatttggaaaatgctttgattcaggaaatggtggtgtttttcgtccttgcactgtttgtatgagagggcgtttaccgaaaacttgggcatcaaaactggcataatcaaatggtacttttccaaacttctcttgttcttttgacactgtggctctgggagaggtgatggcttgtgacgggaaattgaattcaatttgcttcaccaaacttgtcctgtgggcctggtcaggacactgcccagtttggggagaatcaagctgatttttatcctgggacattgccaatttttcagctgcagcaattggacaaccagaaagactcctgtgggtgttgcggttgctgttcacatgaccccttcctgtgcatcccggcgtgggacacttgagcacattttcatgcatggcaagaatttccaggggaacccgcactttgtgggggcaccccgaaaggctgcggtggtgcgggtagagccctgtcacgtgtcccgtgccatcacatccagggatcgggcacttggtctccctcttttcaggccttggtgaatgtttattgttaaagatttgtcttccacccatgtcgataactttggtttgcctcctttcccctgctaggtgctccagcaggaacctatccagctctttgtaggtgttatggaaaacacaacctcgctcagcctgcagagcaattgcctgctccagcaaacttaaattccccttggccttttccaggtcactaccctcttccgtcattactgccaggctctcgctatcttcctcctcaacgtcagggaatgagggctgggcattgccatccaggggttctgcgagagcattctgcgggtctttcctttctgtttcagaatcacacctgttctcacaagggataaatttgtcaccttcagtttttatttcaggaacttccaataggtcttttttatgatctgttaaaacatactttgggactctaggtggtttggtttcttctgagaagttggagccactgtcccagccattttctgcactttcagagttactttcattgtcatcagaggagcagaagggtggctgagaatcatcaatcttgtctcttccatcatcagaatgaatcagaaagcactcgtctgcttcatcgctctctgcttttaaagactggatgccactgtcatttaaattttcacttacagtctgaacagatacatttttttcaaatttccccaagtgcattaaagacttgaccatgagctcttgataacaagagtatctgtcttccttcctactggagttttcttgtgcagttgaaagaagactttcatccataggttttatcatgatttcctctgcggtagagtgaccatgtgtttccaaggggccatcgtcctctgtcctgtcactgcggtcttcttggcagtctgcttttgggctgtagtgtcggggcttcattagcagggatttccttttgttgactggaacccccaaagcctgatcttcagctgttctcttctttgccatggagcaatcataggcaacactgagctcctggattagtgaatccattggcacctcggttcctttagagcgagtacgcagcgttttatcttcagcctctgcatccatcttccctaaaagctactggatctgaactggagagtttccatcactcttttttgtttgtttccaaaacttatatttctctcctccctggtgggctgaacggaaacactaaagctgtttctttgaaaggtagttcccatgatatgac

SEQ ID NO: 18721 - RNA, 1404 nt, Homo sapiens
  source 1..1404: mol_type = other RNA
tgagtgtgtgtgtgtgagtgtgtgtgtatttccatgtacagtcatgtgccacataaagcacttctgtcaagaatagacggcatatacagtggtggccccataagattagaacagagcagaccttgtacaggtgtactgtatttgatcttttataccatatttttactacactgtttctatgtttaggtatgtttacatgcacaaatacttaccattgtgttacaatcacctgcaccattcagtacagtaccaccctgcctgggtttgtagcccggtagcaggaggtcctgccatacagcccaggcgtgtgggaggcgatgagtctgtgccatctaggtttgagtaagttcacactatgatgctcgcacagcgacgaaatcgcctaacagcgccttcctcagaaccatccctgccatcgggcgatgtgtgactgtatgtgtatatgtgtatacacagacatgtacgtgtatacatacagtgcaaaatattgacagttggtgaatctaactgaggggcatgcaagtggtccttgtctattctttcaacgtgtctgtttgctcgaaagtcctcaaggtaagctgggggaaatcatctaaaaggcggcaagaaaggaaagaatttatacacagaatctgcaaacaaacagtatacgtaaaagaaaacagcagctccaaacttagatgtatcagtaattgcattaagtataaacagacgaagagctctacttgtgagcctatgtcgttgactctgtgtgtgtgtgtctgtgcatgtgtgtgtgatggatttgtctgtgtgtgtgtgtgtgtgtgtctgtgcatgtgtgtgtgatggatttgtctatatgtgttttctatttttaaaaagccaacattggcagagcaaatgcagttacctggagctgtccagcaaaggtagcctgatacccagcatcctctgcatgtggcatgttcagggaacgttttctctaaaataactagaagtgcaggtgcatcaggaagtgcagatgcccaagggattctcaccaggaagttgcagatgaaccaagaagtctgcaccaggaagtgcaggtgcaccaggaagtctgcatctgggagtgcaggtgcacccggaagtctcatgtggaagtgcaggtgcaccagaaagtctcatctcccagagcagcagcctggcctctgctcctctccgggcagaaacgacacagggatgctccccagtcagtgtgctggggtcctaggggcgttggcgacgccggggcaggttccaccatagatcctgctgcctcaatccagagggctttcggaaggcgcccctgctatggcatcgcagagggaggagacccgggatgtggcccagcagggctgtgtatacaccaagatgcctccgtctgcccttccagctgtaaat

SEQ ID NO: 18722 - RNA, 3764 nt, Homo sapiens
  source 1..3764: mol_type = other RNA
tgagtgtgtgtgtgtgagtgtgtgtgtctctacccagctctcctacaccttagccccaaggatgatggggagaaaaatgtgggagctgactaggtggaaccaaatctttactccagaaatttatagctaatataaaactcttaaaaatgaaaaaaaaacagttttcttacctttttaaaaagtcttctctttggggggttatgtcaggggatagaggaatgggcttgagccagttttcaaaattgctataggccaggcgtggtggctcctgcctgtaatcccagcactttgagaggccgaggcgggaggatcgcttgagctcaggagtttgagaccagcctgggaaacatagcaatgccctgtctctacaaaaaatttaaaaattagccgggcgtggtggtgtgcgcctgtgttcccagctgctcgggaggctgaggcaggagggtcgcttgagcccagaaggtccagactgcattgagtggagatcgcactactgcactccagcctgaatgacagagtgagaccgtctcaaaacaaaaacaaaaacaaaaaccaaccaaaaaaccaaaaccaactccctccccgcccccgaaacaacaacaacaacaacaaaacccccaaaaaccaaattgctatagaccaatatttccaggtccctgtgattttgattagagagttttgttcttgttcttctgttccgtaaactatggtattctacctcttaaacgcatttttaagctttctagtttggatggccttaaacagagaagcccgtccctgggtggggaggtttgtccgctgtccagtagatggcgctgtgacttctagagtgaggggggtgggggtggggacgacaccgcgtcgcagcccgaagtcacaggggccaccccgtcgcctctcccagggtgtatccatcgggctgtttctgcgccagccagccttcttataatcttgtttatttccagaaatcacatttgtgacagctctaataggccattcaacagcaaagattttctcatttagttgaaaatatttcaggcttcagaaacctttagtcccgtcagtgggggagtgaatcctgcaggatacaccacgtttcacgtcctccccattctccctgcaccccgtgaaattctcttggaaggagatggaaaactgtgggggtttcatttaagggtcagctcacatgtttaagctgcatgtcaggaagaagaaggctgagatcctttgagcaaacaagtgccagaaactgaaacccctgcctgtctcttgtgcaacgcctccccagcggtttggagacttgagcatttgaatgggaggcgtcccaaacatttcagtccagatctcctccaggagagggtgctggggacccaggtctctctctagggctttgaaagaggcttgctcggtggagacagaaaacatgggagcagtccaggggagcagttgggctttcacagagcaaaagctgccatggccatccggttccaggcacttgccatgcagacatgggcatgaggcctagccaggccaggagcttggacagggccacactgctactcagtgacagaggctctcctgaccactccagagcgccatacttttccttggaacgctaatcttggtcattcagtcctttaacaaatgccttagtttttaatttgttaggtgaccatctcccatgactagaatctttgttgtgattgctatattcccagtgccttgagtgatccatgagctgcacttataagaaagctcggtaattatccagagtttacaagggagcgggtgcggcatgggataactcaatgctacctcccaacaagtcaatgaggtaggaaatgtcattactcccatttgacaatcaaggaaactgagtccctgagaggttgagtgaaatttgcaaggccacacagctagtgtggagagttgtggggcaacagggatttgaatccaggctgtcagatcgaggaccacacattcttaactgggcctcatagtgctttggtaaataaatattggttgagtgaataaataagaagatgaaattgaaaaacagtggggtgcgatgtctgcagcgagagtttcagaggagggcagatttgggttcacacaggcctttactctcgtttactgatgaccggtaaattccttaaattttctgagcctcgacagtttcctcctacatgaaatggaactaaccatctttctttctgggttgggaagacttgagcttgtgaatgaaggacttggcccatagcaagtgctgaataaagggctgcattatgactatctctgggccagcccccaaagcccagacgtaagcgggcagaggagctgctgcccgtaacacatctctgactccaaccaactgggtgaccctggtaagtttctcagcttgctgtgtcttgcttttctcttctgtagaggatggctcactcttagttcctgcctggaaggcttgcatgaggaaagggggccaggcccaaagtcagtactgaatgatcgtccacttggaggttcacattaggcacttgtatccttgcggcactcacatgttgggatgcgtggcccactggtggctggcgggaatgcccgcgctcggtcatgcttcggtgcttttgcacacgctggcccttcgccctggagtgtttttccaaccagtgaatctcctttcaccacttaagtgcactgcgtcgctgaagggtaattatctgagtgttccaactctccctcttgccctttctgggctgttctatccgagagcatatttgtcacttagcgctgggtcacctgggttacccatctctctgactgtggagtgtgagggttaactcacgtcatcccagaccaacttggtaaaacgcccctggccacatttccctacggatacaagatgtaagggtgtgacattgtggtagaagaaggcatgagtgtgatagaagaaggcatgagtgtggcaaaaggaagctttgtttctaagatctccaaacccaggcccacgagcggcatccatgcattcactcttgcagctggttgccgttcaatcagcaaggagtatttattgagcacctgctatgtgcccggcacttgagtggctctaggtttaaggctatgaacaagagaccagggcgacccttacccctccacagcttatcagaaggacgacaccgcacgggcgatagcaggcctgggtgtggcaggcttggtggggatggtgggtgtctcaaggaggaagtttcagggaaggctttggagacggggcctctgagctgaggtgcaaaggattagcctggtgtagggacggggcagaggctttgcaggcacggggagtggagggtgcaagaccgcggcgagggggccggcgaggggggcgtgggagtcggggcaggaccctgctggacacctggtctgtcctcagtgccgctttccccagggccacacaggctggctctggttatacccattttacagacggagacactgagatcagggagcaccggtggccctgggaaatggccgggcctgctcgttaatccccaggtgagcgggattcgctggcctggggggctcctctcccaagagaccatctccagggacgtcatagttcatgtcctgagcaagccggcaggctggttttaccaagaaagtaaataggtaaataaaacaagtaatacaataaaacaaagaaaccgatcaacgacatcttgaccttagtatgcccgggtggtctgcttttcggtgtccccaaggagagaggaaat

SEQ ID NO: 18723 - RNA, 23257 nt, Homo sapiens
  source 1..23257: mol_type = other RNA
tgagtgtgtgtgtgtgagtgtgtgtgtgagtgtgtgtgtgtgtgtgtgtgtgtgtgtgtgtgtgtgtgtgtaattcaaggtaaagttttcattattaaagactgcccaataatctctctcaggacactgaagcagaagctagaagatgccatcagagacccagtagccagatgtagctgctgattacgaaagacaggatctacactggctactgagccattgagggtacctacaccttccagcagctgggtgatcctttgccttctggggaggggctctgtggaagaaaaaagaagatatcagatttcaattgcacattttctttggatcatgaattgacattttgacaatattcccatgtacgtaattttaaacaacctctggatttatttacttatccaacagatactgactgagtgacattaaataaagtgccacatattttcttaggtgctggagatccagcagcaaacaaaaaaagtggaaaatctctatacttctacagcatacatgattccttgtgacaaaatctacaatcaattatttggtatgttttgcagtaaaatggaaatatacacaagagaaaaacaaacaagcaaacaaaaaaccaatctaccattttattgtggcttggagcatttttgttgcttcctgtcactttaacttgggtaatctagcaatgatgcacatatgtaaagtaaattgcagttaaaaaattctttcgtgttacgaactgaggataatacagttattttaccaaatatctcaaacaccaaagaaaattacagaaaatgcatattataataaatattcaaagcaggtgctcactagcatgtcagttccaagctttcctcccatgatacaatgaaggtaacaaaataagtcacaggattggtgttctctttgctattcatttatccaccccagaaatacttactgagtaccttcaataagtacctttcagtaccttactgaaatacttctgcgtgctttattccaggcactgggaatgcaacactgaacaaaatccttgcactcacggaagtttaagtctaagatttaaggaaagggtagaaaaagactgaaaaaaacctccatagatatggacggtcatttcatagagtaatgaaacagttaagaggaatgctattttcgataaggtggctaggaaaagcctcactgagggcctggcatttgagtggattcctgaagtaggaggagaagaatcatgtacatacctggggtgggaaaggacaccacagggagaggcaagagtcagaacaaaaagcactgaaacaggaaaaagcctggtatcttggacaaggtgttcttttattagcacatgaccacatggccaattattgtttcctacttttaggattattctagaaggtaaatgactatgcaacttttctccaagtacacgtcttagaatcctttgctgtgaatttaaaatgcttcagctatcacttagaaaagatttaataaagctactgtcaattggaaactagtaccatttgatcggacatgcagctataccacagtatgacacacacatatttatcaccaagagaaaagtggctttttaaaaatgtgttagctataagaaaagataaccagctttctgggagctctaaatatatacatatctagggaatgatttaactatttaatcacagatgtctaattttaagaggcaactcacttgccaaattatagtaatagtgcttcaccagtgtggttagctcttggtgggggaggataagggtggaatttacaaggtgaagcaggggtttttttgattgcttgcttttttttctctttaaataagttaaggccaatcccatctatgaagtatattttggcactgcctacaaaccagagcatacatactgaagtgggggaaaagaccgtttatataggtttggctaagtcttaccctcaatgtaaaataaagcatttgtagaacacacaaacttacatttcataaaccactaaaactaactgttcataactctacttttatgaataagactaacaattaaagtgaggcaagggtttagtgtggtcactttcaatgccaaaatacaaaagattatcttttataaatctttacatttagatgagaaaaggtaaatttttaattctcaaaggtatctattctccacatcttagtactaaagttaaggtggtcttttgccccttgttttaaatttaatctaggtaatacaaataggaaaatctgtaaataaaattttattaaaggttattctgtaaattagtgtcaaccactaaacaatactatacagttttaagtttattaaaaacacaaagaatagaatatgtagaatatataacaccatagaatattaaccaataatgcattttcagtttaaaaataaaaggaaaagaaaagaaataggttcaaactagaaatgttgagttatataattctgttatctaacaattaagatgacaactaagccccaagggtgagtgataggactgtaaccaaggtacttctgctcaagtcctagtcacactgcaaacaaacaaaacaaaaataataataaacaaaaactcccatacattctggctaaagaccatttatttgaggtatgagaaagagtttaaagggagggaaagactattaaaagttaagcctgccacctgctgttggaaggcctgctttgaactgggataaagaccatttcttgaaatgttaacctagaatttgaagagcttacactccacacggttagaacaggggcaacctatacaccaaaccaagaagtaaagaaacccattgatgtttaaagctacactgagagagataaaagtcacattcgcatcaaagttctactggaaatgaaagaaatgctgcttcgtgcgtcattctactgaaggaagagtagaattactctgtcttttaaactgattacctggacaattctattttgcccccaaaaagcatctctgactttagaaattatcatttttagaaagaaattttgaccctagggactatatgtggaagtaaatgaagagagatgaacgatttcacagcattgccagaatgctaactttaccaagtcaaaattgtctaattcactgtttttaacacaaatgtgaaagaatctatgcttctttgagtaaaagaacttccagatgctttccagttccatgattttctataacctcacaaagtctggccccacatgtccccctaaaccccatccatgatatttcacatatttttgttcatgcaccagtagttttctgtaactaaataggaatagagtcaaattctatcacaatcatgtttagggatttgacagagcataagccagtccactattctaatgaagtcagagtttactttagaagtgaacaaaaactgccacccacagtgtatatctcatgttaagtgattcttaacatatacacaaacacagacacaaaaccaaagggatacaatgaaactttgagagatgttgaatacatccattaccttgattatggtgatggtatcacaggtgtttgcatatatccaaactcatgaaattttccacatgaaatatgtgcagttctttatcaattatacttcaataaagctgtttttttttttaaaaaaagctgcctcccacaccgttaagaacaaaaagtccaattaactctaactgtaggccagggaagaaatgcacccatgtatacacagtgcgccacagggtgaaattatgctagaggagaaatcagccttttaaatacaggtgtctaattaaagtatgttcttatgaacttggattccttctgtgttatgttatgttagagcaactgagccagggtatcaccataaccgggcacgtggttgaaacccgtccagctcttgcatacctgagatcctgtgactacactgaccaaaaacatttataccagctgatggtcacttgattctcacatctctctatttagtaaattgctccgcaagccaacttgaagactgaggtgaacattctctgggacgttcctgctgaagacatttttttaaaagacattgcccctgccagataattctagtctgaacaggcctcagaagggactggttggcacaagatcctaaaacaagcttctaaaggtgaaaccactcagagcccataaagacagactcagactagttttttaaaaactaatatttaacaattaggtgcatgcctttaatccttctcaacgaaaaacaacattttttaaacaatcaatagatgaaaacatgaagcattttactcattgcaaacactcagaggaaaaggatagttttaacctaagtaacaaacagtctttttatggacaagtttcagaaattaattgccctaaatccatgtacatatatatctctctttgtccctctccccacactctggaagaaaaccctaaggcattctctacatacaatgtcagcagtgtgcaacgatggtgaggaattcttgtcgtttttaaataaaagaaagaggaaaataatttgcattccatcaatgataagtaaaaacaaaagaaggacgtcaaaataaagtaacttctctgagcttgtgaatagcagaaaaaccagtcagttctctcaagaattcatgacttagagacttatttagtgacaattaacccattactactctatactattaccgaggcctttctgtggatttggtctcatttttaagccttgtgctattttctaaaggcatcaacatcgcacatgtctaccattgcaaccttcatttataatcagatctctaccaagcctctgcttttggcactgtacagaacttcttttgtcatacaatgttcttatggtacaaaattctttgtgtcgtcttccttgaatcttcccatcaagtttccctctcctcagatggactgatggaggagcaaaattcggcttctgaacactgcctgacaagcacttccctccctgcaaggcccagctctcttataggatgctaagggaccttcctggattcctctggaaagttagctgcatactactgggggctggttcccagatcactgagtctgtggtctcagccagaaacacaagacacattgctcttcaatttgtttagaaatgtgtctccctgtgagaatatgtgctctttgagggtaagaatcagtcccataattttgagattccccaggtaccagcatagtacactagatcatagtcaccttttagtaaatatttgtcaaataaagaaatgtgagtgaatagacagtaaaatgcctgacacctatactgatacatttcaaaaaacaacaaacacaaacacacacacacacacagtggaagactatctccattcagggaaactcttgtatttcttcatcctttaaacatttcttgctttctctcttagttttatggtagctttctgtaagatttgtgggtgcttataagatcatgctatttgtaaaagagtgtatgttccttttaacagaagtatggactagtgaaagcactgtcttagagtgtgtttgtgtaccatcacaggtttgtagcacagaagggtcctcagggaaataaaatctactccagtaaaatgataaaactaagacaaatgaacaggtaatgagggaagaccagaaagagaacatccatatatacagtttcttttgcttatgatggttatcagaagctcaaccacattaggtatcaattattatgagttctatgacagtatgtggacttttaaaattaagtggcttatataaatagctcacaccacaatggaagagaaaggaagatagttagcagaagaagtgtgaagattcggaaagactaataaaaatgatttttaaatgatgaagggctaaatgtatttcccgcagatgctatttgatgacctatcaggtacaaaacacacacacacacacacacacacacacacacacacacacttcagcaaagaggaacaggatgaaaacatggattctacttgtgtaacaaagagaaaatggaaacgctaattaagatttttaaagaaagaatgttctaaaatgtgttaaacgaagggaaagaggggaaatagatattttcaaactacgaagaaagactacagtataaagacctaacctacaagtccagtatttgctcccagagtggctgccacacagtggacgtgtgatcagttcttcaacaggttgtaaggaaacctcaactgttttggaggaaataactcggtacaccccaaggaccatgcaaagccttgataatagcacaacagcatccttctaccccttcttctctccttattggttgatgctggactgtatttgtgctgacagtggaaggttttttgacaacgtatggacagttctatagagcaaaatataagtatctagaaaaacaacatcaatataattaaaaatcagattaaaaattaggattcaaaacactaacaaagaggaaaatggcaaaatatcaagcactcagcttacaattggagatggtctacaacatgacagtctggaatgtaaaaaggaagcaggatattgaagagggagcaccaccgcaagtgagaaaagagccagggagagagacgtcagtcaatacaccagaagagaaaatggacatagggaagcccaatgcccagatactcatcaatgaggcaagagcttcatgggcgcccactattattaactaggtagaataagaagtttaccaggtagggaaaaccagaaggtggggaagggaaggaggctgaggagtaactcttggaggtttaaaaaaaatgttagaaaaggtgagcatccggagtccatgacaaagcgaagattattcataggcctgggcaaagtcaagagatgaaggaaggaagtctttcttcctgtgcggggtggggagagcagcagcagcaaactttatcactaggttgaaaggggaaataacagaaacaaaactgctgtttgtattgatggcagtcacacaggggaaatctggttcctctttctatgagtgaagaaagaggtcaggggaggtacttggcactaaaggatgatataaccttgaaaggactggctcagggaggacaagagaatggtgtgtgtgtgtgtgtgtgtgtgtgtgtgtgtgtgtgtgtgtgtgaaggggagacctggtggagtgtgaatggcaatatgctatgggagtcgttttcactcaaaaaggaatagcaaaaccctctcatacagagaaaatgacagggcgcaaggagctcaaaaatgaagaggagccttccacttctaacaagaacacactagatgtaaattggcaatgctgaaagagcagtgagtcccagagccagaaggaactttcctaaggtatccagcccgtggatagtctaaatgtcccacgtagatgtgacaagccaggaatgatcccaatttacctagctccagaattgcctgatcttcttcttgactcaatgcccccaacctcacattcatccccttgcttcccatttctagctagtaggtaacagcactgagcccgttcaaatttctcacagacagtctctattcattctgacattatctctccagtaagtcctactctggttatcaaactttctgtagtctggagaacaaacaaatccctaatatggtcattcttttcatgctgagagatcaaactcatcctattactgggatcagtaatagtaaatgcaaccctgacaccgacaggagagagtcgtcaggtacattaccacttttcttcacagctgcccctatgaatgccatgaaggaccacggaattagggatggaataaattcgaggatttgatgaaaaacaaaacaaaaaaatagggctccctttgattgtcatccttagacaaaatttgatactctttgcactaccatatgattatatcccctgattttctaagattaaagtccattagagttagaaattggaactctcaagccgaagtcaagaaaacaaatcatgtctggttttagaggtgccagaatgatacaatggactttggagacttcggggaaagggtgggaggcgggtgagggataaaatactacaaattggggctgcgcgtggtggctcacgcctgtaatcccagcactttgggaggacaaggtgggcggatcacaaggtcaggagctcgagaccatcctggttaacacggtgaaaccccgtctctactaaaaatacaaaaaattagccgagtgtggtggcgggtgcctgtagtcccagctactcaggaggctgaggcaggagaatggcatgaacccgggaggcggagcttgcagtgagccgagattgcacccctgcactcctgcctgggtgacagagtgagacttgtctcaaaaaaaaaaaaaactaaaaattgggtacagtgtatactgctcgggtgatgggtacacccaaatctcacaaatcaccactgaaaaacttactcatgtaaccaaacaccacctgttcccccaaaaccaacagaaattttaaaaaatttaatttaatttaaaagaaatcaatatatgaaaaaagaaaaaaaaaaaaaaaaaaaagaagtgccagtcgggacagacagagaactctcaggaaaactgctcattttgccaatacatcaaatagttatttaaaaaaaaaacaaaacattttctaaagtgtgttagagggctagtgaagagagaaggccatcgaaaatgatgaagaataaggaggagagatgtacaggcaacacaaccaaggagaaaaggaggatgccagacatgggtcaatcttgttagctaagtaaacctcaatggtatctgcctctaagctctgtttggtgagtctctgggacccaactaatgatggtttagtgtcctttaaagaagaatttaaaataatccagtacataggatttcttattgtgcaactttccaattctgaaggaagctatagggcaactaatgttaactaaactgctatgtctccctgttgggtttgcaaagccactcagtactgtgtgatcagtaacccaggaacaaagagggcagtcacacagtaacatcaacacccactgggtacacagagttgcccacttttcatgactcttccacgtgtaagggtcacaaacttgggaagctggtggctgtgttattacccatttagaaacggggaaacagaggattagagggaattatcatcttgaacatctcatatttttaaaaaggaactctaataactacctgacaaattggtgagtgaagagtcttagccaaacactcaatgacaatagtttgaggaagaagcaaagtgtagtagttagaatggtgatttctgagcaagaagatgggggctctgtattcctggccaagtagcttggcttctctgggtctcagtttgctgccaaagcaaacgaggataatactgatcctacctgtaataggaccattgaaaggatttcacaggatgaggtttatgaaaatactttatagttaataattctacatcatatacctgaaatttgctaagagagaaaaatcttaaaacgttctcaccacaaaagataactatgtgaggtgatacatacgctaattagcttgattgtggtaatcctttcacaatgtatacatataccaaaacatcatattgcacactgtgaatatatacaatttatttgtcaattatacctcaatacagctggaaatacataaattttcatgcactgtgtaaatatgagagatttatttctccaacaatgatagaatctgaaagtggggattttcatgtcttatctttgcaatctgaacacagcaactttggatgtcttagccacattgcacggtagactgctacagtaagtttgtttaagtgctaatgcttagaagtcgggcaggcagctggaaccaccatgctggaaaagatacttcctgaaccacttgttcaaatgctttgtaaacaaaagggactaaagagatcccatttattatgttcactgtttaactttggtttctcatctgtactagaaggtcgtatttctgtcctcaaaccattaaaactctatcaggttcccccctccccccaagaaatgctgattttgccaaataagggcattttaaagccttccatctactataacaatgatttcttattttaagttttttttaagaattaaggaataactgacatacgataaactgcacatattcaaattgtataatttgataagttttgacatatatacacccatgaaaccatcaacacaagacagaaattatccaccagcccggaagttttctcgggcctttttgtaacccctttcttgccacccccatctcccctaccccaggtaaccactgatctgctttcacattttccagaattctgtatacatggaatcatatgatatgactctcatgggttagggtcatccatgttattgaaggtatcaatagttcattccttcttattattgagtagtatccatcatacagatacaccacaatttgtttatccatttacctgttgatagacattaggattgtttccagcttttagctattactaataaaactactatgcatattcacgtacgagtcttcaggtgagcacatgctttcttttctctgggagtgaaacagctgaatcatatgataggtgtatgtttgacatgtttgtatcattttacatgagagttctaaatcctacacatccttaccaacagttggcatggctggcttcttaaattttagccattcagataggtgtgtagcagtacctcactgtggttttgacttgtgtttcactaatgacattgaaaagattttttcttgtgcttatctgccatttgcgtatcttctgtggtgaagtgtctgttcaaatcgtttacccatttttaaattttgttttcttattattgaaaatgccatcagttttaatgagtggagcaagactggtaactgagaactgcaacaaaattttacaattcatgatacccaagaggataaaaaaattcacaaagattattttccaaaacttgtgtggagcgaaaatattctccaaatgttatgacaaatctgaacttcttttaaagcttgaaaaggatttaatgatattttatcagtattgctgctaagtctgcacaggttcagactattagtaaaccaaataagcatatttcgatgtactctatcggtacccaaaccatcttaacctctccttcgtgcattagttcaattacccaagcatctatccctaagccacatttcacactttgcactaattatactctaatcccatagattccattttactaattatttcttatgtcaaatttgtgcccacattcaaaaggtgatgaaggccaaaacctctatcgcatttttttatgtcaacagtaacagataaaatgtgatctacaagcatgaagatgaattctcctttccgatccatagagaatgctagatttgagggcacctacaggctttgaggaaaagcaggccccattcggttgtgtagagccatcggttcgtagctcaattgttacagttgatgtgggtttccttttagatgtctggaaaatgactctgctgaccacatccacattctgaaatactttttgagaacttgtaaccaaactgcaggaactgactcattttgcagtgcccagccaccacacaattgttccagaacagactcaagtcaaagggaaaaatatgaaggtcttagaacacagacagcaagttgtctacttatatggggggacaaccgggggaaatcccagagcacatggggcaaaacggctcaagccccggaccaatcttagaggaaggaccaaacagaactcaccacttcgtggacaacacatgtgttttcctcaaagcaagggggtcagaggctggtagaaaaagaaacttaatgtctatctcttagacactaatctacacttagaaagtagattcagtagagaaatgtctgcagaagactcgggttagatgttgtcttgaaagtccattcctgaattccttgtactcccagctcctctgagatgggatgctcagtaagtcaggagtatgccccttgtcttacaggagataagccagcagggacagcatgtccaagatgctaggcagaactgaggctgacacttgagcttaggaccagaaattctctggctcccctggggcttctgtacatcctctcctggtccatttttacatctttctcttaattcccaatgtgtctcacccaagggggtcagtttccccatgatgtcccaaatctttctccctctctcaatgcagacttcttacctaaggggaggatgaagaggagcaaactaagctctcctccacacaacactctatgttcccaaattactcatttctctaccccacaagtgaaactgatttagtcagtcagtttcagccaaaggcggtgaggaaatccggtcttgttgaactaaactataaatgacaaaaccaataataactcttttctgcaggtgggtcccttgctaaaagaatatgagggttaacccaacccaaatctatcattgactaatagaaaggctatgtgataagaattaggtatagagtctcaggcagtatttcaagtaagataaacctggacgacacctataaaaggctatcaagcccctttctaagccctgtatgttgtcgatataattacatatacattttatgtctgttctcacccgtgcaatgtctcttaacatgtaaactcccagatgacagaacttgcccatttccttagatttagtaaggggcatttagtatccgagtataatagtgaagtaatgacagggggctgcaatcaaattatggcaatcaactctacctttaagaaattacaaaaatgtttttaacacaactttacaagagaaaaggtacataaaacaattttacccttcccacctggccaattgcctttatttttccacactctctttgtacctccaataaaataagtactgtataacaagacttcttaacctgtaccaaacagtaagttttcatacagaattttaaaaaggagcttatcatctgactgaacataaaactaagaattattttaaaatgaaagcactttaaacatggatttaaaatcccttcagttcaaaattctaaactgcttgttactgagtgcaaaaatcagcaaagatatgccttatggaagatgagtttttggcaaatttaaatcaaatcaaaacattccacagttagacattcaggtaccccacatctctctgaggagtagatgtgataggaagaattgcccactttgcgctttttagctgtaattgtgcttcaaatagttcaactttatctatctttgctaaggttttcatagcataataatttaaattacaaaagtagcattttactgcaagaaggccttacacggcttgtaaacactccagttatgaggcacaaggggctcgactctccgggatccctacaataaatcacatagactctcagaataccatcttcactctctctagttatcatttcctaccttccaaacagcttcttactgtggccaacagagtcctacctgatctgccatgatgtgtctcttggacacacaaagcctgctcccgtctctactgcagttacttttttattttctctgcctggaatcctcttcctccagacactcccacagctgattcctcactggcctaataacatcaaagaggccttcctattagccctggttaacgtcgctctacccctgatccccaggtactctctctctgacacagctttatttttctccgcagtgtttactaacacctgccgtatacttatgagttccatcaccatcagcctacccgctccatgtgagcggggactttattcactgctgtattaccagacccagaactctctaaggcacatggtagacatggtagatgtataatatatttttgtaaaatgtacatttcccatgtggtgtcttagtctgttgtgctgctataagcttatgaaatttagttggcacctgagacaatttttgttaacaccttaccaaaactccaaacgcctcaagggccaggtggacaagagctgtaggaaagtgatcactcccccagcagtaaaaaaagaaagcaggaaaaagaacagtttctctataatctccctgctacccatgcatagcaaataagggaaggtcttttggagtatggatgtcaaacggaatggggagaaaggtagatattcactgtcattatcaacctaacttgtcctgaggcctccttattggttttaacacagagagagagaagagccttgaaatactgagacattcttttagagtgtgagtgattttgtttttgtttttaaatctacttcaacattttcttcccttgggccatatatacccactaataatgtagacttcacatttcatgctgaaagacaaagcattttcattgcctttgctggtatggtcaaacttgtttcagaaaatgcacaggtatagtttgtgccattgaagacaacttgaagagtgatgtctttcaaaaactataggaggtgatatcaagatttaaataacaagtaaagataatgactctgtcttaaggaagcgtattcctaactgcaacatggagacgagtaatattttttgaaagaatagtagtataaattccaaaagccctcccctatgttcattcctcattttctatatatttacttagagatattttcaaaaagtcataataaatttgattgagggcatggcaacacttcttacctttaaattaattaaaattctattttaaaattatttttgaagacatctttgtgatggcctttgttgtctcttaatgttcttttattataagcgtaggcaggtgaagcagcaggagtagagaaagaacaaagcaatctgtaactggttgtgatcattaattgtaaacgctactgcacttaatatctttaaacaaggaaattatttgaaagcatgagtgctcttagattatatttactgatacgttccctactatgaacccttcttccgccaacattaaaaagaaagaaagaaaaaccatttctctgcactgtttttccctcacaagcattttctcctctcactttaaaaaaagaaatgcagctcccaaaggaagatgcttaaagaccttcatgagtgttgtgagtgtctgtctgtgaaatatacgttgtctccaaagggacaaacaatcagatacaagatgcagtcagtgaggtgaaaggaacatagagtgagtttattgcttctcctctcccgtcccctgatggactctcactcccatcctttctttcacctatttgcaggtagatgttgaatgacttatgcgagagtatggacaaatgaaggaatgaacaaacaaaggaaagaatgaaggccggcatgattaataaatcctccaagagcaggctcagtccaaggccaggggatttttttttttttttaaagagacttccaagcactctgaacccacgggctaggataacatgccctcatcttctaagtcaaaattctcaatctacatcagaaagaggaaattctcaatgtgaaacccctttcccatattctgaaaattaagtccacacccaaacataaggttttatgcacatagatggcttcctgtacttctttatctagaagttttaccccatcctccagaaaatatccagaactagatggagataaagaagaaaaatattagtaaatacagattcttacacatttcatttttctatggattagttctataccagcaagaaggaatttccagaaaggttgatgtaagtgcatccctaggactcaaatgctaacatacttctccctcccacccccactttcaagtgaaaacattagagaaaaaaataggggaagttacatgattaaacttgttagtatatgagatcaactgaaaacaaggaattcccctcctggactgcagtggcctaattaaaactcataaaacacaaatgactaagactgttcccgttgatttgtgaaataaaaagcagaaaaagttaattttgtatttcaatattgacagaggtaggcctagaagacgtgacactttacagaatagaaatgagaagaccatttccgagactttcaggttcagtcaacttttattctgctttcctgccagaagtacatgtacttaccatctgtactggcaacagcctatttggatttagattctggttccatgacagatgagtggccctaagtaagttcctttacctctctgtgcctctgtgtgttcatctatgaaatgggcatgataattgcaccaatagtttgtcatgaggaaaaatgggtcgatgcaggtagagcccttacaacagtgcctgtccagaacatggtaactgcacaataagcgacagtcaccatcatcagtgttttgcttaatctgatgtgaaaaaaagtcatatcacttagcatggatctacaggctttaggactaaactgaagaagtctgttcctaaagggattttggaagggaatgcaagtgtgttaagcaccattactccaggtcccacagcatgtgctttacatgtgttatctcacacaacaaacctgtgcactacttctgatgctctacactctggggctcagggaaatagcggagtagcttactcagctagcaaggggcaaagggagcttaaagcacaaatctacttatttccaaagcctgggcctcttagggagtaaactacttcaatggaggctgtgaatggacaccctcttggggtcatgggtaccactttcacgcactaacactctctggaaaatgtctgaagctttcaagatttttttcaggtaatccgaactctgaatgttccctgcaaagttttgccgggcgtgtacatatttactgtttctctcaactttaagaactctagtctcacttcagatatattatacaaatcctaatcaagaaaaaaaaaaatcaatggattttcacttttaaaaatctttcttccctctccttttaggaaacgcagaaaaactaagctttctttcaataccaacaccaacaatgggctttcaataccataagcacatcaggggaattaaactcttccatggcagaaagaggagataatttaaaatgaaacctcagcctactcttcatagtctaccttaaatagttatactatgtttttaaaaagcaagttattactttagtaaccatttaaaagaaagtaactagaactattttgttataaagcatagctaagaaaacaaaatgtcccaatcattatattaacttacaaaagcatactaaattcaacttttgtatgtatctaatctgttcctttaagaattagtctaggccaggcgcggtggctcacacctgtaatcctagcactttgggaggctgaggcgggcagatcacaaggtcaggagttcaagaccagcctggccaacatagtgaaaccccgtctctactaaaaataaaaaataaataaataaaaaataaaaaaaaattagccgggcgtggcagtgtgtgcctgtaatcccagctactcgggaggctgaggcaggagaatcacgtgaacccaggaggtggaggtttcagtgagccaaggtcacaccattgcactccaggccgggtgacagtgcaagactctgtctcaaaaaaaaaaaaaaaaaaaaaaaaaagagagagaaaagaaaagaaaaaaagaactaggctaaagaaaaaagatcaactaaaatgatgcatttacataaccacattgtttatagttaataatatatgtgggggtttttttactttatgttttagattgccctaaatatgttggaaagaataaactagaataaatatggggttgaaaaacaagaggttagagttgaggattttaagaacttgagtcaggaaatattcaaggttaaatcacttacagtctttaatgtgtagaataactgtttaataattgatttatttttcaaatgaaaacagtaggaagtaggtaggtttaacaggtcttactcccaaaacatgtcatatacagttacccagttgtctatttaaattgaaggtagttcataaaatgcaagtgtttactttgcatgttctccttagtaacttaatcttctggatttgttacccaatgattatattcaaacttggctcaatttcccctcctgaatgaagacgtctattctccaaattcagactgtataaccagtacagcttgtttaagaaaaataaatatgataactaatagtaaaaaaaaaaaaaaaaggcaaaaaatcatttatttacagcagtctgagattgataggagggaatgagttagaagatgagcatcaaaaagaaataaatctaggacctttaaatgtattcaaagaaaacaatactgctagtgtctaattaaaatgtcaaatgaataaataagtaagacatacaatatgtcagacagaggcaagtgctaagaagaaaaattaagcaggaagaaggatagaaagctggggaatagaatggggaggttgccatcagtttgaaatgaatttttttatccctagaaacatatagggacttgagacatgccttatatacattttttgagaagtactgttaaaggtatccttttgtgaattcaaagagtcatgcagctgaagctccatgggctgcctgatttctgccaagaggctctgctgtgtcccagtgtagttcccaagccagggagctcacaaccttggaggtgacccatgccctctttattgattccacacctcctgctgggtaaggggtctaaggaatgtctacaaaaacgtttttcccactgttcaaggaaacttccttagggttaaggaaagagttatttcctatgtcttaatttttcaagatgaaaaagtcgggctgatttactgatggagatcaccttgggaagcctgtgaggagagttcagacccctggaattcctacactcccacccaggagaacctgttataagcattcaaccacagccccggctaatgaccatagtggtgataccaccagctcttgatcgtaggaggtatagggtgactatgaataaagtaaatcactcaaacaccccctctgactcagttaagaagtccagtgccacatctccagtcctctcttgtacctgcatcagaatcattaagagcagattggagctagactgtctgctttcaaatcttggctccgctacttcctgtatactgtttttgtgagttaaagaatttaataagtgtaaagcagttcctaccaaaacgtgtctactaagtacctactatgtgccagacactgttcttagatgccagtgattcatttagaatggtacccggcatataatatgaactcaatgtatgtcagtaattatgggtccacaaatgcttacctgacactcagattgattattattattattttataaaggtaataggttgactattcaatatagtatataaacctctaggggagtctggaacaatactccgtgatcaaacacattaatacttctacagtaaaacatacaaagattcattctgagcgagctaaacaaagactatcattagcttcacatcagttcaggtcaggatttgctgccaaatttgttacatgaaaatcttttgattttcagagctttttggattacagaagagatggtgggcatatatttattaagagactaaccccactgaaatctttttctttctaacttcaggaggttctagcaaccaaataaatagttaaaactatttaggagtaggaaataggaagaccttcagacatggaaaatcaacaactgcataattaagctatgccaaatattagtctgaacaatccctctcctcaaatacagtgctccatagattctccattgacagacatttccacaaacaacaggtctcaaacaatctttttctaagtacttttcaaaagcactttttgaatatagaataaaatacttaaattttatcactattttaatagtacaaccttgtctttcccatagaaaaaagacaaaagctattaaatgacaaatgaacaactggtttaaaaacatgtgccttaaaagaacacagtatcctctgtagtctgcctgggggagatgaataaacgttatgccaaagtggtaaaccatcctgctaccaaaggaattttctccacattgcattttaaggaaattcacagctcttgaagagctatacaataactggttcaagatgttctcactgctggtcagcactggataaaggatttgcagaaacccatggaagcctatttctcttgcctctttattgcccccatgtgttgttatttatcttccccaacttttctgaccctttccatgtatttttttaattgaagtattgctttgttcaagacctatgtttaccactcccatggcgatcctgtacacaaagacaagtcaggaagacatgaaacgaacggagatacttatgttgcttcatggtttttccccttctcattatcctcctactcaatgagactatagtgggaggtctgaatgacatttccaaaccaagaacttaaagctacatttcaacacccaactactcagttgtcataggaacaacactatgaggcttatctgggttctaacaaacagccacttgtttcactaatgattaaaactcccccttcaaatcaaatatagacacccatacatatacagacctcaaaagaaaaatttaattgggtaaaactgtatactacaccaaaaacttaagaaacaagcccaaagggaaagcatttacgttcccgaacatgcaaattcaaacactatttcagagaaattattttgaggtctgtctcttgaccagatcccttcagtttgttgttttacacacccacaaagacaaaggcatatgcatggcattaatatcttttaacagggtatacgaaaatgtgaatactctcaatgaccccagaggagaattcagagcaagcaatgctactcactttcgatgtacttttaaaaattaacaaattgagaacagagaacggcaaatagaattgaaaacatgaagttctcagttaattcttctgggatatactttctagcatttactgttccaacctgtttctatcacattttgtcattcaaaacaatggattttaaatggatgaggaaaacctaaaaattagaggcttttttccaacaggcacggcagtatttatccagattattaaatcatcatgttctccccaagtatttacttacatgaaatacagagttgaaaacataagctagcagttgaatataaattatctgtaaataccttaatgctttgttgccatttttctgtcttcaagactctaaaaacctataaattcatgtgcttcaagaaaactaatgccattccttaattaagtcaaattgacttgtcatgttcacaagtttggatcacccgtttcctgacttattggaggacctgcccttaagagccgtgcttatcttgtctttctatttctttaagaataaatacttatgcaaaagtcttgagagctgctagtctgagaaaactgatctcaaaagttatccaagtatacaagagggggaaaaaacaattaatatatctcactagattcatctccctcccccaccctcatcccactccactgctaagagagagaaatttcagcactgctatcctgttttattatacattttcccttttgagttaaggattttaagattttgaaagtaacagaacaggaaccaaaagtagattcaacttccaatttggcttaaaaagaaagaaataattattatttcctatattacccaaaacttattctgttaataacagttataattatatattcaaattaataaatgaagattgctaaaattgcctatatacttgttagcagttaaagaagaaaaattttttccatttgcttctataagtagacatcacatgattacttctattgaccaataagaaactagtaaaatcaggcagtcacccaccattcttttctaatgttctttttcttattctattcaaccttttcagtatattcttaagaagccaaatcaagaaattagacattcatgcctaaaataaaattgcgttaccttatacatcatgaacaggaacctgttgtatataacacgggtattcaaagctttattgtctttttctagaaccctttaacataaaggcagctcagattcaagattagaaaactgaattcaacaggcaggaacacgcatacgaaaccagtaagaactactaatcacgacctctcaaaatgtcatgaaccatatagatagaaataaccccccttttgctgtactaatgtaatccaatagaacaaacttaaaattcgtgacacaaatgtaagaaacaaaaaacaaaaatctattgccattgtaatctacccttcccaatcaggagaggtgtttccgacgcattacttgaactttcattttgtacaactttcatcttgtaaggttctaactaaatacttgacatcttaatgcagaggaaaggaaaggagggcaagtagactaattctgaaagcatcccttcaaatttcatacatgctattcagactaaatggaaatctacatccatggaaagttaatgtcgcaattctactaaacagcccattctgattttatgtttctcctccactaacaagaaaaaataaaacaaccaaatctagctgtattacatatgtttagctaaactgatagcactcagctcatttttgttaattacctggcttcttctcagtctttatgcggtattctcgtgctgctcttttttagaactcctcactgtttatgtgttctctgttcaacacagttgttaggggtctgtgaacaatttttcaattcccacacacgcatatgatatctattagggagcaatgccacttttcacttaccaattctggataaaggagtatttcctggtgacagaatgctgctgcttccgttcactaaaactccctcttcgcagcttgataaatctgattataaaacgtctttgttccagatcacacgaggcgcttttcctacaaaagttttctaaagagttatctgcatttcattccagttcaggaagcctagagtttgatcaagtcggtcacaaccactttgagagtcttccactggtgtgcggactccaagaaagcagtcacttggtcatctatcacatgtggctgaatcactggacagaccacccccgccccacacacccccagcccccgttgagcagcagcccaggcaggagagt

SEQ ID NO: 18724 - RNA, 2111 nt, Homo sapiens
  source 1..2111: mol_type = other RNA
tgagtgtgtgtgtgtgagtgtgtgtgtgcatgagtgtgtatttgtgcatgtacgagggagtaagatcactcaaaggtgaaggggtcctgggtgctgaaaaagaagtgtccatccatgtggtcctccagggcatccttgtcactctcagcaggaaagcgctccttacagataggacactccttccatgtgggggtggcagggcccccagtgctggtttctgacagggtacccactgtaaagccactggccatgtcatagaaggcactgcccagttcaggaagcagtaagttggcctcctcacccccactctgcacagctgccatcaggactgacttctcatcttcagcctccgagtcagagctactgtcctcagctggcccagagaggtgaggagaaatgggagccggctggctgatgacaacaaggggagaagcctctcgaggcccagcaggagaggagcctgggtctccacgctcacaaaggccatagggtgggagcctcatgtcttctggggactcgtcctctgagtctgtcagagctgccgggcagctcagccccacagcggcctcctcatcctctgtggtggcatcctcattccacttctcatctgccaccttctccaggcgggcctctagctttctcatgtactctagcaattcctgtttctcctcctgtaactgctccttttccttctggagcacacgcagggctgaccgcagctctgtcagctcccgcttactttctgacaactgtaccaggctagaatccttctcccgggccagctcagtcttgaacacttggttttgggtcctctcctcctgaactgccttctccaatcgaagtatctctgcactcagcttcaggatcttgtccttctctgcctccacactctgcagcagccctgcccgctccttgctccattggcatttttcttccttcaagtgcaaaccgagctcagccagcctgccgttaacttcagccacttccaggcggctgcggtgtagttcggctatggtgcggtccctggctgctgctgcactggccaactcctccccaagaagggtggctttctgctggcttgaggctgcaagctcctgggcccctcgaagctgctccttcaagggctccagctcggccacccgctgctgggcctggcctagggtgtccttcatctgggccaccttgtctttcagtcgctgagcctgagcactctgctcctcttgccagctcttcgcctccttcaggtccaaatttaagtgatggttctcctgttgtgccacttggagctcagcctcactttgctccttgtctgcttgtacttctttcagttgcccaaggagcttctcttgttcccgagtcagggccttcactgtgtctctaagcctgtccagctccacttccttcgtcagcactttctcactgatggtctggatgtcatcctctagctccaggatgcgtgccacatggtctccctgttgccggctcaggatgtccctctcttctgtgatctccccatgggaccgggaaatccccttgtactgttccatcagctccgtgtgctcctgcctggcagttgccagagccctctcgagctcctgcactcggctcctcagctctgtcacctgtccctccagctgtagcttcagctgcatcaggtcattccgttcttgctggctctcatcgagctggttctgtaacacagttgccttggggacaaccagcaggatgtcagagcccccatcagcctcctccagggtcaccagttcatccatgggccttggctctcggaactggaaaggggggctctgcccacacacctggccctggcggttcacatatcggaactggtagagctgagctcctggtttgggcaggtagctggcttgaagatgccaatccagtcactggcactgggcatggtgcctgggggaagggtgtagtgacattccaccttggtgttggggatgtaggtccgggctacattgagaaagttgactccaccacgggatggtgcccggcttagtggtgattcttccatcctggccttgagatatctgtcctcccaacagacggatcagctgttcccctcacctttcaccaacaacaaaaac

SEQ ID NO: 18725 - RNA, 2214 nt, Homo sapiens
  source 1..2214: mol_type = other RNA
tgagtgtgtgtgtgtgagtgtgtgtgtgcatgagtgtgtatttgtgcatgtacgagggagtaagatcactcaaaggtgaaggggtcctgggtgctgaaaaagaagtgtccatccatgtggtcctccagggcatccttgtcactctcagcaggaaagcgctccttacagataggacactccttccatgtgggggtggcagggcccccagtgctggtttctgacagggtacccactgtaaagccactggccatgtcatagaaggcactgcccagttcaggaagcagtaagttggcctcctcacccccactctgcacagctgccatcaggactgacttctcatcttcagcctccgagtcagagctactgtcctcagctggcccagagaggtgaggagaaatgggagccggctggctgatgacaacaaggggagaagcctctcgaggcccagcaggagaggagcctgggtctccacgctcacaaaggccatagggtgggagcctcatgtcttctggggactcgtcctctgagtctgtcagagctgccgggcagctcagccccacagcggcctcctcatcctctgtggtggcatcctcattccacttctcatctgccaccttctccaggcgggcctctagctttctcatgtactctagcaattcctgtttctcctcctgtaactgctccttttccttctggagcacacgcagggctgaccgcagctctgtcagctcccgcttactttctgacaactgtaccaggctagaatccttctcccgggccagctcagtcttgaacacttggttttgggtcctctcctcctgaactgccttctccaatcgaagtatctctgcactcagcttcaggatcttgtccttctctgcctccacactctgcagcagccctgcccgctccttgctccattggcatttttcttccttcaagtgcaaaccgagctcagccagcctgccgttaacttcagccacttccaggcggctgcggtgtagttcggctatggtgcggtccctggctgctgctgcactggccaactcctccccaagaagggtggctttctgctggcttgaggctgcaagctcctgggcccctcgaagctgctccttcaagggctccagctcggccacccgctgctgggcctggcctagggtgtccttcatctgggccaccttgtctttcagtcgctgagcctgagcactctgctcctcttgccagctcttcgcctccttcaggtccaaatttaagtgatggttctcctgttgtgccacttggagctcagcctcactttgctccttgtctgcttgtacttctttcagttgcccaaggagcttctcttgttcccgagtcagggccttcactgtgtctctaagcctgtccagctccacttccttcgtcagcactttctcactgatggtctggatgtcatcctctagctccaggatgcgtgccacatggtctccctgttgccggctcaggatgtccctctcttctgtgatctccccatgggaccgggaaatccccttgtactgttccatcagctccgtgtgctcctgcctggcagttgccagagccctctcgagctcctgcactcggctcctcagctctgtcacctgtccctccagctgtagcttcagctgcatcaggtcattccgttcttgctggctctcatcgagctggttctgtaacacagttgccttggggacaaccagcaggatgtcagagcccccatcagcctcctccagggtcaccagttcatccatgggccttggctctcggaactggaaaggggggctctgcccacacacctggccctggcggttcacatatcggaactggtagagctgagctcctggtttgggcaggtagctggcttggaactggacactggtgtgaatgggggaaccatcagttgtactttcaggcacggaagaccacacaaatgtgtggtaatcccgaacacaggcagcctccaccttgaagatgccaatccagtcactggcactgggcatggtgcctgggggaagggtgtagtgacattccaccttggtgttggggatgtaggtccgggctacattgagaaagttgactccaccacgggatggtgcccggcttagtggtgattcttccatcctggccttgagatatctgtcctcccaacagacggatcagctgttcccctcacctttcaccaacaacaaaaac

SEQ ID NO: 18726 - RNA, 2352 nt, Homo sapiens
  source 1..2352: mol_type = other RNA
tgagtgtgtgtgtgtgagtgtgtgtgtgcatgagtgtgtatttgtgcatgtacgagggagtaagatcactcaaaggtgaaggggtcctgggtgctgaaaaagaagtgtccatccatgtggtcctccagggcatccttgtcactctcagcaggaaagcgctccttacagataggacactccttccatgtgggggtggcagggcccccagtgctggtttctgacagggtacccactgtaaagccactggccatgtcatagaaggcactgcccagttcaggaagcagtaagttggcctcctcacccccactctgcacagctgccatcaggactgacttctcatcttcagcctccgagtcagagctactgtcctcagctggcccagagaggtgaggagaaatgggagccggctggctgatgacaacaaggggagaagcctctcgaggcccagcaggagaggagcctgggtctccacgctcacaaaggccatagggtgggagcctcatgtcttctggggactcgtcctctgagtctgtcagagctgccgggcagctcagccccacagcggcctcctcatcctctgtggtggcatcctcattccacttctcatctgccaccttctccaggcgggcctctagctttctcatgtactctagcaattcctgtttctcctcctgtaactgctccttttccttctggagcacacgcagggctgaccgcagctctgtcagctcccgcttactttctgacaactgtaccaggctagaatccttctcccgggccagctcagtcttgaacacttggttttgggtcctctcctcctgaactgccttctccaatcgaagtatctctgcactcagcttcaggatcttgtccttctctgcctccacactctgcagcagccctgcccgctccttgctccattggcatttttcttccttcaagtgcaaaccgagctcagccagcctgccgttaacttcagccacttccaggcggctgcggtgtagttcggctatggtgcggtccctggctgctgctgcactggccaactcctccccaagaagggtggctttctgctggcttgaggctgcaagctcctgggcccctcgaagctgctccttcaagggctccagctcggccacccgctgctgggcctggcctagggtgtccttcatctgggccaccttgtctttcagtcgctgagcctgagcactctgctcctcttgccagctcttcgcctccttcaggtccaaatttaagtgatggttctcctgttgtgccacttggagctcagcctcactttgctccttgtctgcttgtacttctttcagttgcccaaggagcttctcttgttcccgagtcagggccttcactgtgtctctaagcctgtccagctccacttccttcgtcagcactttctcactgatggtctggatgtcatcctctagctccaggatgcgtgccacatggtctccctgttgccggctcaggatgtccctctcttctgtgatctccccatgggaccgggaaatccccttgtactgttccatcagctccgtgtgctcctgcctggcagttgccagagccctctcgagctcctgcactcggctcctcagctctgtcacctgtccctccagctgtagcttcagctgcatcaggtcattccgttcttgctggctctcatcgagctggttctgtaacacagttgccttggggacaaccagcaggatgtcagagcccccatcagcctcctccagggtcaccagttcatccatgggccttggctctcggaactggaaaggggggctctgcccacacacctggccctggcggttcacatatcggaactggtagagctgagctcctggtttgggcaggtagctggcttggaactggacactggtgtgaatgggggaaccatcagttgtactttcaggcacggaagaccacacaaatgtgtggtaatcccgaacacaggcagcctccaccttgaagatgccaatccagtcactggcactgggcatggtgcctgggggaagggtgtagtgacattccaccttggtgttggggatgtaggtccgggctacattgagaaagttgactccaccacgggatggtgcccggcttagtggtgattcttccatcctggccttgagatatctgtcctcctactcctaagcttgttgacccagctgtatccaggaatgagttatgacatcagaaagcagcaactaatctccaacagacggatcagctgttcccctcacctttcaccaacaacaaaaacagcactccgacttctggaggggagggagaagagtgggcgcgagggcttctggggtttgtggttcttct

SEQ ID NO: 18727 - RNA, 2392 nt, Homo sapiens
  source 1..2392: mol_type = other RNA
tgagtgtgtgtgtgtgagtgtgtgtgtgcatgagtgtgtatttgtgcatgtacgagggagtaagatcactcaaaggtgaaggggtcctgggtgctgaaaaagaagtgtccatccatgtggtcctccagggcatccttgtcactctcagcaggaaagcgctccttacagataggacactccttccatgtgggggtggcagggcccccagtgctggtttctgacagggtacccactgtaaagccactggccatgtcatagaaggcactgcccagttcaggaagcagtaagttggcctcctcacccccactctgcacagctgccatcaggactgacttctcatcttcagcctccgagtcagagctactgtcctcagctggcccagagaggtgaggagaaatgggagccggctggctgatgacaacaaggggagaagcctctcgaggcccagcaggagaggagcctgggtctccacgctcacaaaggccatagggtgggagcctcatgtcttctggggactcgtcctctgagtctgtcagagctgccgggcagctcagccccacagcggcctcctcatcctctgtggtggcatcctcattccacttctcatctgccaccttctccaggcgggcctctagctttctcatgtactctagcaattcctgtttctcctcctgtaactgctccttttccttctggagcacacgcagggctgaccgcagctctgtcagctcccgcttactttctgacaactgtaccaggctagaatccttctcccgggccagctcagtcttgaacacttggttttgggtcctctcctcctgaactgccttctccaatcgaagtatctctgcactcagcttcaggatcttgtccttctctgcctccacactctgcagcagccctgcccgctccttgctccattggcatttttcttccttcaagtgcaaaccgagctcagccagcctgccgttaacttcagccacttccaggcggctgcggtgtagttcggctatggtgcggtccctggctgctgctgcactggccaactcctccccaagaagggtggctttctgctggcttgaggctgcaagctcctgggcccctcgaagctgctccttcaagggctccagctcggccacccgctgctgggcctggcctagggtgtccttcatctgggccaccttgtctttcagtcgctgagcctgagcactctgctcctcttgccagctcttcgcctccttcaggtccaaatttaagtgatggttctcctgttgtgccacttggagctcagcctcactttgctccttgtctgcttgtacttctttcagttgcccaaggagcttctcttgttcccgagtcagggccttcactgtgtctctaagcctgtgattggtgggatgacatgtcagacaatctgctccacccagagaaggaatggactcaggcctctgtcttgtgctctgctgctgctgctctaggcccagagctccatttcactctgggatgcataaatccccaagccagctgatccagttctaagccccaggaaaccaagattccaggttctgtccagctccacttccttcgtcagcactttctcactgatggtctggatgtcatcctctagctccaggatgcgtgccacatggtctccctgttgccggctcaggatgtccctctcttctgtgatctccccatgggaccgggaaatccccttgtactgttccatcagctccgtgtgctcctgcctggcagttgccagagccctctcgagctcctgcactcggctcctcagctctgtcacctgtccctccagctgtagcttcagctgcatcaggtcattccgttcttgctggctctcatcgagctggttctgtaacacagttgccttggggacaaccagcaggatgtcagagcccccatcagcctcctccagggtcaccagttcatccatgggccttggctctcggaactggaaaggggggctctgcccacacacctggccctggcggttcacatatcggaactggtagagctgagctcctggtttgggcaggtagctggcttggaactggacactggtgtgaatgggggaaccatcagttgtactttcaggcacggaagaccacacaaatgtgtggtaatcccgaacacaggcagcctccaccttgaagatgccaatccagtcactggcactgggcatggtgcctgggggaagggtgtagtgacattccaccttggtgttggggatgtaggtccgggctacattgagaaagttgactccaccacgggatggtgcccggcttagtggtgattcttccatcctggccttgagatatctgtcctcccaacagacggatcagctgttcccctcacctttcaccaacaacaa

SEQ ID NO: 18728 - RNA, 1959 nt, Homo sapiens
  source 1..1959: mol_type = other RNA
tgagtgtgtgtgtgtgagtgtgtgtgtgcatgagtgtgtatttgtgcatgtacgagggagtaagatcactcaaaggtgaaggggtcctgggtgctgaaaaagaagtgtccatccatgtggtcctccagggcatccttgtcactctcagcaggaaagcgctccttacagataggacactccttccatgtgggggtggcagggcccccagtgctggtttctgacagggtacccactgtaaagccactggccatgtcatagaaggcactgcccagttcaggaagcagtaagttggcctcctcacccccactctgcacagctgccatcaggactgacttctcatcttcagcctccgagtcagagctactgtcctcagctggcccagagaggtgaggagaaatgggagccggctggctgatgacaacaaggggagaagcctctcgaggcccagcaggagaggagcctgggtctccacgctcacaaaggccatagggtgggagcctcatgtcttctggggactcgtcctctgagtctgtcagagctgccgggcagctcagccccacagcggcctcctcatcctctgtggtggcatcctcattccacttctcatctgccaccttctccaggcgggcctctagctttctcatgtactctagcaattcctgtttctcctcctgtaactgctccttttccttctggagcacacgcagggctgaccgcagctctgtcagctcccgcttactttctgacaactgtaccaggctagaatccttctcccgggccagctcagtcttgaacacttggttttgggtcctctcctcctgaactgccttctccaatcgaagtatctctgcactcagcttcaggatcttgtccttctctgcctccacactctgcagcagccctgcccgctccttgctccattggcatttttcttccttcaagtgcaaaccgagctcagccagcctgccgttaacttcagccacttccaggcggctgcggtgtagttcggctatggtgcggtccctggctgctgctgcactggccaactcctccccaagaagggtggctttctgctggcttgaggctgcaagctcctgggcccctcgaagctgctccttcaagggctccagctcggcctcactttgctccttgtctgcttgtacttctttcagttgcccaaggagcttctcttgttcccgagtcagggccttcactgtgtctctaagcctgtccagctccacttccttcgtcagcactttctcactgatggtctggatgtcatcctctagctccaggatgcgtgccacatggtctccctgttgccggctcaggatgtccctctcttctgtgatctccccatgggaccgggaaatccccttgtactgttccatcagctccgtgtgctcctgcctggcagttgccagagccctctcgagctcctgcactcggctcctcagctctgtcacctgtccctccagctgtagcttcagctgcatcaggtcattccgttcttgctggctctcatcgagctggttctgtaacacagttgccttggggacaaccagcaggatgtcagagcccccatcagcctcctccagggtcaccagttcatccatgggccttggctcttggaactggacactggtgtgaatgggggaaccatcagttgtactttcaggcacggaagaccacacaaatgtgtggtaatcccgaacacaggcagcctccaccttgaagatgccaatccagtcactggcactgggcatggtgcctgggggaagggtgtagtgacattccaccttggtgttggggatgtaggtccgggctacattgagaaagttgactccaccacgggatggtgcccggcttagtggtgattcttccatcctggccttgagatatctgtcctcccaacagacggatcagctgttcccctcacctttcaccaacaacaaaaac

SEQ ID NO: 18729 - RNA, 2291 nt, Homo sapiens
  source 1..2291: mol_type = other RNA
tgagtgtgtgtgtgtgagtgtgtgtgtgcatgagtgtgtatttgtgcatgtacgagggagtaagatcactcaaaggtgaaggggtcctgggtgctgaaaaagaagtgtccatccatgtggtcctccagggcatccttgtcactctcagcaggaaagcgctccttacagataggacactccttccatgtgggggtggcagggcccccagtgctggtttctgacagggtacccactgtaaagccactggtggttggggaaggggtagaggcaggagagaggggaagcagggcaatttgggctctgcagaagatggtgctggccatgtcatagaaggcactgcccagttcaggaagcagtaagttggcctcctcacccccactctgcacagctgccatcaggactgacttctcatcttcagcctccgagtcagagctactgtcctcagctggcccagagaggtgaggagaaatgggagccggctggctgatgacaacaaggggagaagcctctcgaggcccagcaggagaggagcctgggtctccacgctcacaaaggccatagggtgggagcctcatgtcttctggggactcgtcctctgagtctgtcagagctgccgggcagctcagccccacagcggcctcctcatcctctgtggtggcatcctcattccacttctcatctgccaccttctccaggcgggcctctagctttctcatgtactctagcaattcctgtttctcctcctgtaactgctccttttccttctggagcacacgcagggctgaccgcagctctgtcagctcccgcttactttctgacaactgtaccaggctagaatccttctcccgggccagctcagtcttgaacacttggttttgggtcctctcctcctgaactgccttctccaatcgaagtatctctgcactcagcttcaggatcttgtccttctctgcctccacactctgcagcagccctgcccgctccttgctccattggcatttttcttccttcaagtgcaaaccgagctcagccagcctgccgttaacttcagccacttccaggcggctgcggtgtagttcggctatggtgcggtccctggctgctgctgcactggccaactcctccccaagaagggtggctttctgctggcttgaggctgcaagctcctgggcccctcgaagctgctccttcaagggctccagctcggccacccgctgctgggcctggcctagggtgtccttcatctgggccaccttgtctttcagtcgctgagcctgagcactctgctcctcttgccagctcttcgcctccttcaggtccaaatttaagtgatggttctcctgttgtgccacttggagctcagcctcactttgctccttgtctgcttgtacttctttcagttgcccaaggagcttctcttgttcccgagtcagggccttcactgtgtctctaagcctgtccagctccacttccttcgtcagcactttctcactgatggtctggatgtcatcctctagctccaggatgcgtgccacatggtctccctgttgccggctcaggatgtccctctcttctgtgatctccccatgggaccgggaaatccccttgtactgttccatcagctccgtgtgctcctgcctggcagttgccagagccctctcgagctcctgcactcggctcctcagctctgtcacctgtccctccagctgtagcttcagctgcatcaggtcattccgttcttgctggctctcatcgagctggttctgtaacacagttgccttggggacaaccagcaggatgtcagagcccccatcagcctcctccagggtcaccagttcatccatgggccttggctctcggaactggaaaggggggctctgcccacacacctggccctggcggttcacatatcggaactggtagagctgagctcctggtttgggcaggtagctggcttggaactggacactggtgtgaatgggggaaccatcagttgtactttcaggcacggaagaccacacaaatgtgtggtaatcccgaacacaggcagcctccaccttgaagatgccaatccagtcactggcactgggcatggtgcctgggggaagggtgtagtgacattccaccttggtgttggggatgtaggtccgggctacattgagaaagttgactccaccacgggatggtgcccggcttagtggtgattcttccatcctggccttgagatatctgtcctcccaacagacggatcagctgttcccctcacctttcaccaacaacaaaaacagcac

SEQ ID NO: 18730 - RNA, 2437 nt, Homo sapiens
  source 1..2437: mol_type = other RNA
tgagtgtgtgtgtgtgagtgtgtgtgtgcatgagtgtgtatttgtgcatgtacgagggagtaagatcactcaaaggtgaaggggtcctgggtgctgaaaaagaagtgtccatccatgtggtcctccagggcatccttgtcactctcagcaggaaagcgctccttacagataggacactccttccatgtgggggtggcagggcccccagtgctggtttctgacagggtacccactgtaaagccactggtggttggggaaggggtagaggcaggagagaggggaagcagggcaatttgggctctgcagaagatggtgctggccatgtcatagaaggcactgcccagttcaggaagcagtaagttggcctcctcacccccactctgcacagctgccatcaggactgacttctcatcttcagcctccgagtcagagctactgtcctcagctggcccagagaggtgaggagaaatgggagccggctggctgatgacaacaaggggagaagcctctcgaggcccagcaggagaggagcctgggtctccacgctcacaaaggccatagggtgggagcctcatgtcttctggggactcgtcctctgagtctgtcagagctgccgggcagctcagccccacagcggcctcctcatcctctgtggtggcatcctcattccacttctcatctgccaccttctccaggcgggcctctagctttctcatgtactctagcaattcctgtttctcctcctgtaactgctccttttccttctggagcacacgcagggctgaccgcagctctgtcagctcccgcttactttctgacaactgtaccaggctagaatccttctcccgggccagctcagtcttgaacacttggttttgggtcctctcctcctgaactgccttctccaatcgaagtatctctgcactcagcttcaggatcttgtccttctctgcctccacactctgcagcagccctgcccgctccttgctccattggcatttttcttccttcaagtgcaaaccgagctcagccagcctgccgttaacttcagccacttccaggcggctgcggtgtagttcggctatggtgcggtccctggctgctgctgcactggccaactcctccccaagaagggtggctttctgctggcttgaggctgcaagctcctgggcccctcgaagctgctccttcaagggctccagctcggccacccgctgctgggcctggcctagggtgtccttcatctgggccaccttgtctttcagtcgctgagcctgagcactctgctcctcttgccagctcttcgcctccttcaggtccaaatttaagtgatggttctcctgttgtgccacttggagctcagcctcactttgctccttgtctgcttgtacttctttcagttgcccaaggagcttctcttgttcccgagtcagggccttcactgtgtctctaagcctgtccagctccacttccttcgtcagcactttctcactgatggtctggatgtcatcctctagctccaggatgcgtgccacatggtctccctgttgccggctcaggatgtccctctcttctgtgatctccccatgggaccgggaaatccccttgtactgttccatcagctccgtgtgctcctgcctggcagttgccagagccctctcgagctcctgcactcggctcctcagctctgtcacctgtccctccagctgtagcttcagctgcatcaggtcattccgttcttgctggctctcatcgagctggttctgtaacacagttgccttggggacaaccagcaggatgtcagagcccccatcagcctcctccagggtcaccagttcatccatgggccttggctctcggaactggaaaggggggctctgcccacacacctggccctggcggttcacatatcggaactggtagagctgagctcctggtttgggcaggtagctggcttggaactggacactggtgtgaatgggggaaccatcagttgtactttcaggcacggaagaccacacaaatgtgtggtaatcccgaacacaggcagcctccaccttgaagatgccaatccagtcactggcactgggcatggtgcctgggggaagggtgtagtgacattccaccttggtgttggggatgtaggtccgggctacattgagaaagttgactccaccacgggatggtgcccggcttagtggtgattcttccatcctggccttgagatatctgtcctcctactcctaagcttgttgacccagctgtatccaggaatgagttatgacatcagaaagcagcaactaatctattcttctctccagactgtgcctgcagcaggactagaaacctactggtttcactttagtatttctctcctcattttctctctgctcccctcagcctccatccttccatctgtttgtattggtagctggag

SEQ ID NO: 18731 - RNA, 2424 nt, Homo sapiens
  source 1..2424: mol_type = other RNA
tgagtgtgtgtgtgtgagtgtgtgtgtgcatgagtgtgtatttgtgcatgtacgagggagtaagatcactcaaaggtgaaggggtcctgggtgctgaaaaagaagtgtccatccatgtggtcctccagggcatccttgtcactctcagcaggaaagcgctccttacagataggacactccttccatgtgggggtggcagggcccccagtgctggtttctgacagggtacccactgtaaagccactggtggttggggaaggggtagaggcaggagagaggggaagcagggcaatttgggctctgcagaagatggtgctggccatgtcatagaaggcactgcccagttcaggaagcagtaagttggcctcctcacccccactctgcacagctgccatcaggactgacttctcatcttcagcctccgagtcagagctactgtcctcagctggcccagagaggtgaggagaaatgggagccggctggctgatgacaacaaggggagaagcctctcgaggcccagcaggagaggagcctgggtctccacgctcacaaaggccatagggtgggagcctcatgtcttctggggactcgtcctctgagtctgtcagagctgccgggcagctcagccccacagcggcctcctcatcctctgtggtggcatcctcattccacttctcatctgccaccttctccaggcgggcctctagctttctcatgtactctagcaattcctgtttctcctcctgtaactgctccttttccttctggagcacacgcagggctgaccgcagctctgtcagctcccgcttactttctgacaactgtaccaggctagaatccttctcccgggccagctcagtcttgaacacttggttttgggtcctctcctcctgaactgccttctccaatcgaagtatctctgcactcagcttcaggatcttgtccttctctgcctccacactctgcagcagccctgcccgctccttgctccattggcatttttcttccttcaagtgcaaaccgagctcagccagcctgccgttaacttcagccacttccaggcggctgcggtgtagttcggctatggtgcggtccctggctgctgctgcactggccaactcctccccaagaagggtggctttctgctggcttgaggctgcaagctcctgggcccctcgaagctgctccttcaagggctccagctcggccacccgctgctgggcctggcctagggtgtccttcatctgggccaccttgtctttcagtcgctgagcctgagcactctgctcctcttgccagctcttcgcctccttcaggtccaaatttaagtgatggttctcctgttgtgccacttggagctcagcctcactttgctccttgtctgcttgtacttctttcagttgcccaaggagcttctcttgttcccgagtcagggccttcactgtgtctctaagcctgtccagctccacttccttcgtcagcactttctcactgatggtctggatgtcatcctctagctccaggatgcgtgccacatggtctccctgttgccggctcaggatgtccctctcttctgtgatctccccatgggaccgggaaatccccttgtactgttccatcagctccgtgtgctcctgcctggcagttgccagagccctctcgagctcctgcactcggctcctcagctctgtcacctgtccctccagctgtagcttcagctgcatcaggtcattccgttcttgctggctctcatcgagctggttctgtaacacagttgccttggggacaaccagcaggatgtcagagcccccatcagcctcctccagggtcaccagttcatccatgggccttggctctcggaactggaaaggggggctctgcccacacacctggccctggcggttcacatatcggaactggtagagctgagctcctggtttgggcaggtagctggcttggaactggacactggtgtgaatgggggaaccatcagttgtactttcaggcacggaagaccacacaaatgtgtggtaatcccgaacacaggcagcctccaccttgaagatgccaatccagtcactggcactgggcatggtgcctgggggaagggtgtagtgacattccaccttggtgttggggatgtaggtccgggctacattgagaaagttgactccaccacgggatggtgcccggcttagtggtgattcttccatcctggccttgagatatctgtcctcctactcctaagcttgttgacccagctgtatccaggaatgagttatgacatcagaaagcagcaactaatctccaacagacggatcagctgttcccctcacctttcaccaacaacaaaaacagcactccgacttctggaggggagggagaagagtgggcgcgagggcttctggggtttgtggttcttct

SEQ ID NO: 18732 - RNA, 2393 nt, Homo sapiens
  source 1..2393: mol_type = other RNA
tgagtgtgtgtgtgtgagtgtgtgtgtgcatgagtgtgtatttgtgcatgtacgagggagtaagatcactcaaaggtgaaggggtcctgggtgctgaaaaagaagtgtccatccatgtggtcctccagggcatccttgtcactctcagcaggaaagcgctccttacagataggacactccttccatgtgggggtggcagggcccccagtgctggtttctgacagggtacccactgtaaagccactggtggttggggaaggggtagaggcaggagagaggggaagcagggcaatttgggctctgcagaagatggtgctggccatgtcatagaaggcactgcccagttcaggaagcagtaagttggcctcctcacccccactctgcacagctgccatcaggactgacttctcatcttcagcctccgagtcagagctactgtcctcagctggcccagagaggtgaggagaaatgggagccggctggctgatgacaacaaggggagaagcctctcgaggcccagcaggagaggagcctgggtctccacgctcacaaaggccatagggtgggagcctcatgtcttctggggactcgtcctctgagtctgtcagagctgccgggcagctcagccccacagcggcctcctcatcctctgtggtggcatcctcattccacttctcatctgccaccttctccaggcgggcctctagctttctcatgtactctagcaattcctgtttctcctcctgtaactgctccttttccttctggagcacacgcagggctgaccgcagctctgtcagctcccgcttactttctgacaactgtaccaggctagaatccttctcccgggccagctcagtcttgaacacttggttttgggtcctctcctcctgaactgccttctccaatcgaagtatctctgcactcagcttcaggatcttgtccttctctgcctccacactctgcagcagccctgcccgctccttgctccattggcatttttcttccttcaagtgcaaaccgagctcagccagcctgccgttaacttcagccacttccaggcggctgcggtgtagttcggctatggtgcggtccctggctgctgctgcactggccaactcctccccaagaagggtggctttctgctggcttgaggctgcaagctcctgggcccctcgaagctgctccttcaagggctccagctcggccacccgctgctgggcctggcctagggtgtccttcatctgggccaccttgtctttcagtcgctgagcctgagcactctgctcctcttgccagctcttcgcctccttcaggtccaaatttaagtgatggttctcctgttgtgccacttggagctcagcctcactttgctccttgtctgcttgtacttctttcagttgcccaaggagcttctcttgttcccgagtcagggccttcactgtgtctctaagcctgtccagctccacttccttcgtcagcactttctcactgatggtctggatgtcatcctctagctccaggatgcgtgccacatggtctccctgttgccggctcaggatgtccctctcttctgtgatctccccatgggaccgggaaatccccttgtactgttccatcagctccgtgtgctcctgcctggcagttgccagagccctctcgagctcctgcactcggctcctcagctctgtcacctgtccctccagctgtagcttcagctgcatcaggtcattccgttcttgctggctctcatcgagctggttctgtaacacagttgccttggggacaaccagcaggatgtcagagcccccatcagcctcctccagggtcaccagttcatccatgggccttggctctcggaactggaaaggggggctctgcccacacacctggccctggcggttcacatatcggaactggtagagctgagctcctggtttgggcaggtagctggcttggaactggacactggtgtgaatgggggaaccatcagttgtactttcaggcacggaagaccacacaaatgtgtggtaatcccgaacacaggcagcctccaccttgaagatgccaatccagtcactggcactgggcatggtgcctgggggaagggtgtagtgacattccaccttggtgttggggatgtaggtccgggctacattgagaaagttgactccaccacgggatggtgcccggcttagtggtgattcttccatcctggccttgagatatctgtcctcctactcctaagcttgttgacccagctgtatccaggaatgagttatgacatcagaaagcagcaactaatcttggtttcactttagtatttctctcctcattttctctctgctcccctcagcctccatccttccatctgtttgtattggtagctggag

SEQ ID NO: 18733 - RNA, 2440 nt, Homo sapiens
  source 1..2440: mol_type = other RNA
tgagtgtgtgtgtgtgagtgtgtgtgtgcatgagtgtgtatttgtgcatgtacgagggagtaagatcactcaaaggtgaaggggtcctgggtgctgaaaaagaagtgtccatccatgtggtcctccagggcatccttgtcactctcagcaggaaagcgctccttacagataggacactccttccatgtgggggtggcagggcccccagtgctggtttctgacagggtacccactgtaaagccactggtggttggggaaggggtagaggcaggagagaggggaagcagggcaatttgggctctgcagaagatggtgctggccatgtcatagaaggcactgcccagttcaggaagcagtaagttggcctcctcacccccactctgcacagctgccatcaggactgacttctcatcttcagcctccgagtcagagctactgtcctcagctggcccagagaggtgaggagaaatgggagccggctggctgatgacaacaaggggagaagcctctcgaggcccagcaggagaggagcctgggtctccacgctcacaaaggccatagggtgggagcctcatgtcttctggggactcgtcctctgagtctgtcagagctgccgggcagctcagccccacagcggcctcctcatcctctgtggtggcatcctcattccacttctcatctgccaccttctccaggcgggcctctagctttctcatgtactctagcaattcctgtttctcctcctgtaactgctccttttccttctggagcacacgcagggctgaccgcagctctgtcagctcccgcttactttctgacaactgtaccaggctagaatccttctcccgggccagctcagtcttgaacacttggttttgggtcctctcctcctgaactgccttctccaatcgaagtatctctgcactcagcttcaggatcttgtccttctctgcctccacactctgcagcagccctgcccgctccttgctccattggcatttttcttccttcaagtgcaaaccgagctcagccagcctgccgttaacttcagccacttccaggcggctgcggtgtagttcggctatggtgcggtccctggctgctgctgcactggccaactcctccccaagaagggtggctttctgctggcttgaggctgcaagctcctgggcccctcgaagctgctccttcaagggctccagctcggccacccgctgctgggcctggcctagggtgtccttcatctgggccaccttgtctttcagtcgctgagcctgagcactctgctcctcttgccagctcttcgcctccttcaggtccaaatttaagtgatggttctcctgttgtgccacttggagctcagcctcactttgctccttgtctgcttgtacttctttcagttgcccaaggagcttctcttgttcccgagtcagggccttcactgtgtctctaagcctgtgattggtgggatgacatgtcagacaatctgctccacccagagaaggaatggactcaggcctctgtcttgtgctctgctgctgctgctctaggcccagagctccatttcactctgggatgcataaatccccaagccagctgatccagttctaagccccaggaaaccaagattccaggttctgtccagctccacttccttcgtcagcactttctcactgatggtctggatgtcatcctctagctccaggatgcgtgccacatggtctccctgttgccggctcaggatgtccctctcttctgtgatctccccatgggaccgggaaatccccttgtactgttccatcagctccgtgtgctcctgcctggcagttgccagagccctctcgagctcctgcactcggctcctcagctctgtcacctgtccctccagctgtagcttcagctgcatcaggtcattccgttcttgctggctctcatcgagctggttctgtaacacagttgccttggggacaaccagcaggatgtcagagcccccatcagcctcctccagggtcaccagttcatccatgggccttggctctcggaactggaaaggggggctctgcccacacacctggccctggcggttcacatatcggaactggtagagctgagctcctggtttgggcaggtagctggcttggaactggacactggtgtgaatgggggaaccatcagttgtactttcaggcacggaagaccacacaaatgtgtggtaatcccgaacacaggcagcctccaccttgaagatgccaatccagtcactggcactgggcatggtgcctgggggaagggtgtagtgacattccaccttggtgttggggatgtaggtccgggctacattgagaaagttgactccaccacgggatggtgcccggcttagtggtgattcttccatcctggccttgagatatctgtcctcccaacagacggatcagctgtt

SEQ ID NO: 18734 - RNA, 5331 nt, Homo sapiens
  source 1..5331: mol_type = other RNA
tgagtgtgtgtgtgtgagtgtgtgtgtgtacacctatacacatatacaaatgtaaatatatgttgaattcatgtttataaacaagttttttaccatgtgaaatatgtactttttcaagtaaaaaataaatactatatcacatctgactctagtagagctgataacatagtgtgggcagacaccaagcagaaatcattttaagagtttaaaaaatcagtttgttttactctaccccaaagaatttcatatccagaaacttcctataaaattgttaaacttatctatgtgtctaatggatgctctgttagatatttcaattgtctaaataggtagctgccaatctggagagatgaaagtaggtaagttgtacttactgaacagctaggttgtatttaaaaggtggggaaaaggggaatgtcttggtagctttatctcaccagtagaaacaatacagtaggtagttacaggcagcttcataggaccaggtggtccatcttggcctgcagctccagggagaccttgttctcccacaggaccagggatgccccgaagaccttctggaccaggctttcctgcaggtccctgaggaccgactgggccggtttttccaggaggaccttctgcacctgcttcccccttagcacctttttcaccttgtcttccctctgcacctgcagctccaggaggacctcgttttccaggaggacctggtgggccagcctcaccagatgggccaggaggacccggttgaccaggatctccatcttcacccttgtcaccaccaacaccatcttgacctgcagggccaggttccccaggaggaccaggatctccaggaaaaccaacaggacccgggttacccttagggccatcatcacctggtggccccttggcacctggaggtccagcagctccaggtggaccagcttcccctttctctcctctttctcctttgggaccgcctacacctgcttccccaggaggccctgggttccctgcttctccaggttcacccttttctccaacaccaccaactgaaccaacagaccctgggggtccttgtggtccatcagctccattgggaccttgagggcctcttgggcctggaggaccaggtggccccatgggaccaacatccccattttcacctttttcaccaggtgggcctggcagaccctgaagacctattggaccaggaggtccagggaagcctctggcaccctcatcacctttttgcccaaacatcccctgctgtcctctaggacctggttcaccatcacctccagcaattccaggggcaccaactggtccttgaagacctgggggaccgggagggccattttctcccttgtcacccttgctgcctttttgtcccggctcaccaatttcacccttgtctccgtcttccccaggggagccggcaggaccagctggccctgggagaccaacaggaccttgaactccatctctccctgcaggcccttggggacctttttctccaggagcacctttctctccagctggaccaggaggaccctgaggtcccgggcgccctggtaaaccaattgggccagctgtacctgctgacccacgttctcctggtgagccaactggacctggtgggccctggggaccttcccctcctttcagtccaggtgcaccctgagctccaggaagacctctttcccctgggaaaccacgtaatcctgctggtccatctttccctgagataccttgaggacctggatcaccctttgcaccttcttttcctgcagcaccaggaagaccttgctcaccaggagggccaggagggccaggatgcccacgttcccctattggaccagtctcaccggttggtccctgtggtccaaccactccccctggcccaggagggccggtcttgccttgaaatccagtctccccacgttgcccagggtgtcctggcagcccatccttcccaggtggtccaggagggccttttggtccagggaatccaactggaccctgaggtccttgaggacctctttcacctggagggccaggagggccatcgccacctgaagtgccctttggcccaggtttcccagtgggacctcttgcacctcttgaacctcgaggacccgttggaccacgctgaccccgagggcctggtttgccagctactccccgtgcacctttctctccattggcacctggaaacccagggaatccagtggaaccctttggaccttgtcttcctggatatcctggtaatcctggaactccaagttttcccttttctcctgcttgacctgaaggacctgggtctccagttgggcctgctcgacctttgggtccttcagggccatcttcccctcttgggccaatttgaccaacttctcctctgtcaccttttagacccatgtcacctttgaatcctggaaaaccatcttcacccttttcacctttagatcccttgagacctctgacaccatctgctccctttactccccgggggcccgggtatccaataggaccttgtggaccagggggacccagagcccccttttctccagactggccttctttcccaggatgaccaggaggcccatcagcaccaggaagtccagcaagtcctggttttccttgtggtcctttttcaccaggaggaccaattggaccttgtggaccaggaagaccctgaggtcctggattcccttgttgacctggaggcccaggctccccttggggacccatgttcccttttggtcctggggggccatctacacctgccataccaggctgccctggagctcctggagttccccttggacccagcaaacctcgtgggccagcttcacctggaagacctcttggtccaatttctccatcttctcccctcattccatcatcaccaggaggacctggaggaccttgaggacctcgttcacccctgtgacctttgtcacctggcagacccggaagtccatcaaaccctcgatctccctttgccccaggttctcctggcattcctcttcctccatctgcacctggacgacccctttttccaggttttcccgttggaccagggggaccctggacgcctcgagggccctgaggacctggatcaccactctcacctttggccccagatgaaccaggcccccccacaggacctggtcttccagttagacccattgggccaggtgggcctctcagagcaatccgagcctgctgaagaatagcttgagcctgagcttcctgagcagagatggttggtcctttggaaccatcaccaccataacggaacggtaacatcaacatagtaccaggaggaccaggtagaccatcagcccctggtaagccaggacgtcctggggggcccctatcgccagggtcaccagggggtccagtggggccttgtagacctggaggacccataatacctgcaggtcctgctggtcctggtggtccttcgacaagcataccaggctcaaccactgctggttctcctttctgtcctttctctccatatgcaccatggccatttatgcttgtttctgtaatatcagtttctgctggtacacctggaccaaattcttcattaggggggcttgttggtttatcttcatattctttatattcataaaaatcatattcgcctaaatctccatctaccagaagatcagaatccctgccgtctatttctttgttttcatatagtgtatcctcagaatttttcctctgggaatcataatcctctcccgttagatattcttcagtaaatatttcttcaactggatttggctcatttgtcccagaaacatgcctaggagcttctgtctggtaactttccattgttccatagttgtattcttgaaaatcatcaacgatgtttgcctttacccctagtttggcttttgctgatgcttgataacttttcttcttcttggatgaaaatttttcagatttggggggtgtaaactttttggatttttcctttgatttagtagccactgtcctcatcttctttttgaaattggatttctttttctccgtctgtgctattgtctcctcagttacagtgggtccctctgttacactttcagcctctttatactctgcttccccatactcatagtcatattcgattatatcctctggtgcatactcatctatctgaggttcctgagcttgagcagccttgggtgctgaagagtcacagtctggactataatgctcacagtagtcatatgctgccttgggatcacctgtgatcaaaaactgctgaatgtccccctcaaaaacttcttcatccaaaatccttgttccaaaaaccgtgattccattggtatcaacaattgctctctcacttctatcaagtggtttcgtggttttcttcttacaatcaacaatcattgtcacagttttcttctccacgctgattgctacccgatgccacttcccgtcagcgatgttaacagttctgaagaggggatagtcttctggggcaggttttccagtgtggtcttcaaacagaaaaacaggtgatctcccaacctcaacaccaatttgctgaataccatgctcattatatatagataaaaggaaagactgaattcctttttttggttttactgtaaatagtattgaaaagtcttctgggaaagttccacctggaaataactgttttgttggggcactgagttgtgcttgctttgaaactctgtaagcagtatctgagcctttagaattctttctgtttgtgcaaaatcccgttgtttttgatattccctctggagaattgtgaaaatctagtgcttttagtacatcaactggagcagctcctctgacctctctagcttggaagaggaaggtcaatgcgagggttgttacggtgaaatcccagagccaccgtttcgttttccacctagaggaccacggctccatctccgagccccgcactcacaactgtgaactcaacccacgaaattgcgactgcagaccaacttcgtcctttccaaggtatcgccagggatgtttgctacacagccattggggagggagagggggaaaaagtcaaagggctttttcttctaaatttgatggtttgcgttcttcgtgtctctagccctttcctctccctctgagttggccccaccggccgggaccctccggccgcgaccctctgatccttcctctgccgggccctgccttcagaatgaaggcagatgaggggcttccaccaacaagctgagagtactgtgtgcccctaaaggcttcatgccgtcagtgggctggacgagtggctccgggcagccccctcctccgcccactcccctccctgctccc

SEQ ID NO: 18735 - RNA, 2296 nt, Homo sapiens
  source 1..2296: mol_type = other RNA
tgagtgtgtgtgtgtgagtgtgtgtgtgtgagagagaaggaaaactagcaacagccatcctacactcctcttatcataacatatgtgtttcaatatttactttattatgagttttacaccttctgaaccagtgtacttaatacaaaagtaggaaaattcatctggaatgaaaaaaacaacagctacaacaaaaagtcactttgatgaagcagcagcccaggctgagtctattatgtatacagtttcagaactgcaaaagagataacgtaaaaaccaggtatggcaaatgatttgagggtcaatctatgtttgtttttatatcccttgctcccacagaagactgtgaacatgtcaagtattaaggacctattttgaattactaaatagacgagatcattaccattagcaaaaattagcaccaaaggatgtataatgagaattattttggcccactaccacccaccaaaaggttggagtttctatatctgtgaattttgcagctctgcagagcttatgaaaacctgctcattttgtcattaacacaagccctactccttagtacttgggggactttgaacatgttcttaacttttccatttccaggttcttccctagtagagcaaggataacagcaatgtccttatttgtaggatccttaggattatggaagtaagctcctggagaacacgtagccagggcatggttccctgaaaaggatctattagtgtgtgctattcttactgttcttatttctgcagtccttgccacatcactgctaccaggactccttcatgaaggatggagtccaactcccaggcacgtgtggatagggtaggggttggcctgctttggtaaagtgagatgataacagatcacacagcaagacgggctgcggacagagaagaaaatccgaacctatagtcagaaagggtctggttccacttgctaaattctgtctcttatcaaaagacaggttttgaaaattattgcaacagaattatcagttatgtgagctttgagagttcttcatttaaaaagatacctcagatattcttaattaatccattttgtgtcttgccattttgttctgtaatttccttgctcatctgattgtgggtgagatttgtaatgaactttctgatacataactatattataccgttttaacgctgctgataaaggcataccggagacttggcaattaacaaaagcaagaggcttgattagactcacagttccacatggctggggaggcctcacaattatggcagaaggcaaggaggagcaagtcacgtcttatgtggatggcagcaggcaaagagagagaatttgtgcagagaacctcccatttttataaatcatcagctctcacgagactcattcactatcacgagaacagcccaggaaagacttgcctccatagttcaatcacctccccccaggctcctcccacaacacatgggaatcatgggagctacaattctagatgagatttgggtggggacacagccaaaccgtatcaatgactccagaggtttttcacagttcacttgattttcaaaatttaataaaaactaggatacaaaaaggcaggctatctgggaactttcataatgatcccttaaaatgtacacatcttctcatggtgtgcctgccatggcgtgcaatttgacctgacagttttcccaggagctaaagcgctgagttttctcctacatggagcttgagtaaccatacagtaggccacccaggtgcttggttttcctttcacacttaagtatccagtgaagagctttctctaatctatgccttctgttcttatgagctatgtctattgaaatgtttggcttataccagaggagggcaataaaataggcaacttttcttcgcaataggacctgagggccacctttttctaccataaagttaccttgcaattctgttatttttgtctctttatttttgtatccatcaatgaaataaaaagcattactctatcatatcatgtatcactgctatagtagacaagaaggaaacattcattcattaaatcttcgaagtagaattttcttatataaatgcatattcttcaagaacaacataaaatgcagcaggtatatgattctttaaaaatacaaataatacaggctattatcgatgttttgttttgttttttctttttctattttagccctgcttaaaggttcttaaggcttcccagctcatcttcccatttcctatctttactcatttatctggaaggaaaattcattcttccttcacagctatgtcttga

SEQ ID NO: 18736 - RNA, 794 nt, Homo sapiens
  source 1..794: mol_type = other RNA
tgagtgtgtgtgtgtgagtgtgtgtgtgtgagtgtgtgaaagtgtgtgtttcaaaggagacttctgggatgatggcgtaaatgtgtatgtgagtgtgtatgtgtttcaagggagatttctgggatggtgtcatgaatgtgtgcgtgtgtgtgtgtgtgtgtgtgagggttcgtgagtgtgtgtgtttcaaggaagatttctgggatggtgttgggaatgtgtgtgagtgtgtgtgtgtgtgagtgtgtatgtgtttcaagggagatttctgggatgatggtggtgtgaatgtgtatgtgtgtgagtgtgtgtgtttcaagggagatttctgagctgacagtggtgtcaatgtgtgagtgtgtgtgcatgtgagtgtgtgtgagtgtgagtgagtgagagcatgtgtgtgtgtgagagtgtgtgtgagagtgtgtgtttcaagggagattcctgggctcgggctcttggacattgggcagaaggctgtgtcctctcctttgaccagtctctgttgtgtttcttccctgagctcatcaagagcagcctcagccatcccaagagcccccagagctgtttgtgggcagctgagcctgtgcagcccagcctcacccttgtcacagtgggccctaccaccatgtttggcccccatgagccatggcattttcacagtcaccctgcatagaaccaaggctggtcaccctttcacagatggagacacaaggaggatgtagcagtagggtgagatcagatcacgaggcggcttttgcttgttttttgataagaaagttttattt

SEQ ID NO: 18737 - RNA, 585 nt, Homo sapiens
  source 1..585: mol_type = other RNA
tgagtgtgtgtgtgtgagtgtgtgtgtgtgtgagtgtgtatgtgtttcaagggagatttctgggatgatggtggtgtgaatgtgtatgtgtgtgagtgtgtgtgtttcaagggagatttctgagctgacagtggtgtcaatgtgtgagtgtgtgtgcatgtgagtgtgtgtgagtgtgagtgagtgagagcatgtgtgtgtgtgagagtgtgtgtgagagtgtgtgtttcaagggagattcctgggctcgggctcttggacattgggcagaaggctgtgtcctctcctttgaccagtctctgttgtgtttcttccctgagctcatcaagagcagcctcagccatcccaagagcccccagagctgtttgtgggcagctgagcctgtgcagcccagcctcacccttgtcacagtgggccctaccaccatgtttggcccccatgagccatggcattttcacagtcaccctgcatagaaccaaggctggtcaccctttcacagatggagacacaaggaggatgtagcagtagggtgagatcagatcacgaggcggcttttgcttgttttttgataagaaagttttattt

SEQ ID NO: 18738 - RNA, 8934 nt, Homo sapiens
  source 1..8934: mol_type = other RNA
tgagtgtgtgtgtgtgagtgtgtgtgtgtgtgtatttaatgaaagcctcattatatactttagtttatgccttcttgttactgagcttagttttcttcgtactgggtggaaaaagaattattttggtttggattattgtttctgaatagtcatgcaattgatacagagatattctggtttgagttcagagctaaaacagtaagtagatacttttaactaaaaacaaatgttaacaaaaaacttagattccctaataactaaagtaaaattcttatgaacaacaatgtgaaggtgggagaattactgagtttccacgtcacataaaagaaaaacacagtaaattctggattgtgctattctccatagagttcccgtaaatactttatcctagttacatgtaaaagttacaaatagcatttgtaaatcaaaataatgatgacaataataataaaataaaaaacactcacttatctttttaaaaaatcaatcgtgagggttttctgagtgcccattttacctgtgagatatggaaggagatgatggaaccatctccattgatccatctctcctttcagctcaggagggcttcattcttctcagctattctcctgcttaaaacctaggcttccagggcaacccatacctctagggccttatcataagctttctacattcacacattgattcatatcttaaaactatgtaattgttttagtcatcgaagtgtgtgtgtaagggtgagtttgtgtgtgtgtgtctgtgtgtgtccacatgaacacatatattaaatatgaaccctctgactggctgcatccagtggcgtgttgaagcatttttgcccaggcttgcaagagccaactgcgtgcatctctttccaaccatgtgttcagtgacatcacagttggtagcttaaaatcatctaaagtggtagtatttatgccatggaaattggcaaatggtgcaaaccaggtgctttctattctcagcgagctggttgttaaacattttaccagcacaccactggttgcatgctaggctgaccaaatgagaagctagatcttgttctgggcaacacggcattaacttagcctcgttggagtgtctccaattttgcttactgtccagggtctccttcctcccaatttcataaacactgcagaaccacaacagggcttgagcatctggggtgcatttgactacccattgtcaccacattgggctctattctcagagacactttcgtagccacatgagtgatgcaggacaaaaccaaaaaggtaaagcatctgaaattccctccgaatatgacagctggcttcctgctgcagagactggagaacaatgagttccccaataggaacaaactattcccagctgaaagcatcagctggggcattcttcaggaggcttcccacagctggtctgcatgctgctgctcaccagcaactgctggcaggcaggcgagcttgagcttgctactgcagcatcctgtcaggggcctggacgtaggcttccttcacttcccccttccctcctcaaagtctgatacaaatcacagagccaacaaaattgaggtcactggcaaaagagtttgaaattttgaatgatttttattaaacaccattagtctacactgcacagttaatgaaacagcaaagctccaatctcttagaagaatgatgactgatcatggatctaaaaagcagttcagtgtcccctaacccaatgtgagcactatgaataattctttaacatctcatgtcagacgcaaaaaggggcaagaactgcaatctggctttgtggggcttccccaccccccacccccccgcccccacccccaccccctttctgccctccccacaatgcaattttcttttagctggtagattacagagtaaaatgtgatgattttggtaaagagggcttctatatttctgaggaggaggatggaaagagaattaatactttttccttcaccaaaaatatcagatggtaggattaatgtctgagaccggcctatctgattagtctcctgccagggtaaatgctgattatgaatacacagatgccacttctgttgttggagtctactaacactaaagagaaaatgaattagattttaattatgagaataaggccgtgcgagtgaaaatgagaaacaacaacaacaataacaacaacgatgaagaatttagtctgccagtcatgtaacagaacactgacaactggctcaataatttttccccacagaattaaatttgggggtgctgaattgacccattcatttgatactgtgtagctgtatcatcttgccacacatttttctcaatggggatagtgatgcttctctaagcaagcagttcattgctttactgagtagtcttacccagtgatccagtttggttctcccacctgccaactcatgcaggtgaattttatcatgtctgttgagaagtatgtgaggcttcaccctcacaactcaactgattctgccttcaaagatattttccaacctcaaactccaacttcaacctccgggatgcaaatttgcatgaaacagaatccaaattagatatctttgggaaagatatgctagaagagtatctttccaatgcagacaaaatctaatgaatttagtgatgtaatgtccaaatgaaaattcatccatttggaaactcaacaaaacacatttttagccaatggtttctaattttgcaacttgctttttgcctgaagattttggtcttttcatttccttacatggaaaaaaaggcatcccgaccttaagtcttttaaaagtagtagcagctaatctgcttttccaattatgtcatccaaatataaaactactagtattttcccaatgagattattaagtaattaacagtctacaggctggctaacaacatgcttacagctaaattctacccggaggaccacactagtaaacccttttcaaagtaatcctacctaccaaactcagacagttatatgacaaaaccactaaaaatccaaagttaattaaaaatacaaagccaagccaacatcataacacaaacttgtcaaactctctgtggttggagcttgggtgacaagtgaaggcgtagtggtggccctacctgggtcaagttgcagggctgagatcatttggtgtacttgctcagatggagcttccttttactctgccctctattctaacctccacgtgcttatttaagtgtgtctcaccaagcctccatcaagatctagaggcacgatctctcactgccatccacatgtctcatatccctcccacaaactggtatactgaagagattcatttgacagaatatctccatcccttagtccctcaaatagctgcacacctacgacacgcatcaccatttacactgtgatgaacagagtaactataaaacagcaacaatccttaatcatgaaactgaaagatgtcttatctcaagggataggaaggtaattcatcctccatgtttaattagttcctaagctgctttataaatgagtctactacataatcaagtggtgatccagagctcgattgtcagatttggtcactgtgctgcagacttggcacatattttacactcagtcaccagagatgacagagaatcctcttgcctccctgttgtatgtaagtagatataacaagtcactgaaactagaactacaagtctttcatccatgaggcaatatgcttgtttctctgggaaactgcctcaacattctaatgtctagtttctggatgtgggatttcaagaagaatctactcctaaatccatgatggtctaggattgtggtttaggttgaacttacaagtcaagccagtgggcttcattatatagtaatagccaggcactctacctggtaaaccatgataaagagacaacttgagtcactgcaaagtcatcagcttaatttttatatgtgacaccaaccttgggtgttcagagtctttaatgttatcatcattttcctcttttaagaggctcagaaaagattctttcaggtttcatttgtgagtgtttggatgcataagtgttgttgctgagactgtaaacataaagctcaaccacagtgggagcataaaaagtgctgggttcagctgcagggatgctcccatcagccatattaacaacatggcttcagccattggagtacaacttccacagccttatacaacaaaaggccttaaactcaaagatgaccagagcacagctcaagtctggctgttttgcaactggggatatatctaaccttgacaatgagagtgcagagtcatcacctgctgtttctatcatggacctgcatggctggctttaataatcacacaagtttgcatctttcatgtgcatatctattatttatctggtcataactcagtgaacagaatttgataacccagcatattaaaggctacatggaattatataccagcaggtaattaccagtaagtaatgcatggatagtgtttaccccaagtgtaagaatcttctggtgagctggaacatcaaaaatgatatttacattgtgatgtttagggacataaaatgaatgtgaaggatcataagggggtagtcacaaccagtgagaaatgtctccaaattaggtgaatggttcccaatgtttagggctctttcaaagcatctcaaggtgaagcactaccccacgactcattttaaaaaaataaaagttagctactatttagagagtttggagttttcttagaaattttcatggaaatgattcacaataatatggactttaataaaaggagtaattgtaattcagtcaaaagttaatgagccaaacaaaggaaagggaaacacagataagagaaaaaagaaagtagaaaacagaaaacctataagagagaaaatgtgaataataattgaggaagtccagattttcaagccactaggaagaaaactgtatatcattacttctaggtagtgataccttgacttttgttcccatagatttgagcaaaatacaatttaaaaatcctgccagttatggacccacttaccaactgtgtaaatgttgttgttgcaaaggaggcagaggtgtgaattccttgttggacactttccagacctctcttaactcccacttgtaagtctagagtgtagcattttggctactaaggcatgcatcaaccaaactgttcttcaaaaggacagctttgcacacagagaaccccaggtgaggatttacacttcaaataatggagttgaaaaacactgatgccagctgatgcctaaaacttgtcaaaataaatgtcaccctttcttcttatcattaaaattaacaaaatagggaatcaggaaagggatgctaacaagaaagtcctctggttgtgtggcatagcatctttttaagagtagcattgctatgctcatttattttcttgatactcttgattttatgatgttgctacaacatctaaccagtgggttttgacaatgaaaattctcacctgaagattgaatctgtgggatacacaaaagtttgacagattctgaaatatgttcttttctgggtataagagtagagtttgggggatggtcccttgtgtctaagttctcatgtatatgtaagaccacttgttgcatttctcaggagcctgtctttatcacaagtgcttcccattctttgttttgggtagtgtgggcttaaaacaatattgtagggactgtcattccataaagcacaaaaagatggtggaatctgagaaatgcatatcaaatgctaaaagaaaaaaaatgactaagtaataaaacgtacactgcccttaagttgtagtgtcaacttacaatgacttctgttttttacagataacaaaagaagcataaaaacaaacataaccaaagagaacgttccccagtgagtggagttccaccagtgaccatcagtgcgctggtagaggtagagtgatgggtcgtgatgctagagatctgagaacacccactacaacaagtgggcatcgatgcgcagccaacacagtccttggcgaacgtagcggacaagattggtcatgctgctgtgctgggtcagaggccccatcagcgtgtccagatcaccaaagaattctttgttttctcttgtcagtttgtcggccatatcccagtgttcatagccccgtaacacattgctagtgatgttgacgtggctggcagccatgtggtgaatgcgctggggaatggtgactgggccattgttacagttccccattgcgttgatgggggagacgttgttgagagacactggggatggagtgttctttccattgcttacccatggagagggtatctgtgcgacttttgaagcattttgcttaaaatattccatcagtgatctggagtacttcatagcatggtccttcttcagcttaaacattctcaaatagaggagtgataaacatcggtagcatagtactgctagctttttgtccccatccgaagccaagggacttgcaaagttcttcagcctcattgcatacctgaggagctccacagtctcagagtacatggtgtatggggactttgcttccagagggtcgcgttccatggcattgccacattcagtgaaggagagggcggcatcagcataattcacagctttgccaaatttctcgaacagtgcatcagctttgtgcttcagcttcttagcttcttgcatgtaataatcagcattgtgaaccgagtcatcaaaagtgagcttgggtctccggacattagtgctgctgctggatagaaggggcagagccgcccaggacgtcatctccaggtgactgctatccatgaggccagtagtgatggtagaggtgatggtggaaatggtagtggtagtagttgtggtggtggccgtggcggtggcagtagctgtgacagtggtggtgacaatggcagtagcagtgacagtagcagtggcaatagcagtattggtgacagtgatggtggcagaggatgccttttttggagtgtctccctcatttaccgatatccctttgaaagtagcacagaatttgccttcagttctcttaggtttggtagatgtgatttgtccagtcatggcgatgtttttgtcttgaccaaagggaccattattgccactgacatttctgcggcgtggagggtcctctggcagtggggaaagtggaggaggaaatagtttttcttcctttcttctatttgctctcctggatgaattattttctctagtgttgggaggcttgtggggtggggctggtgagatgcaaggagggagcaagcagatagttgtggcctcctccaggcgctgcttcttctcagggatcttctctgcaacttctattggcttgtgcttacgtttgcccttaggggctggtttctccacagctgtgacagctgtctgacgcttgggttttgtggcagtctccttgtggtctggcttggcaggtgctgcatggagtgagctgtggccaggtactctagagagtaagtcaaggtcaatcttcacccagaggtttttcaggttctcatgatctcgcagaggggacaggatttcagtttgcatgacaggaataggtgaaaatgttggctcttcattactgatggataagttgttgttgctgccactgctactcattaaggtgctgagggtcaggctggcaccacagatttccttggatttggcagtattacctccagaaataatgcacggaggcaggactttgatttgcagggtctcttcctgatctgtgttggagtcagatgtagatgaatctgtttcaatgaattcccgagactttggcacaatcttgccaggccctctgtacttcttcttctcgggagccaaagggatgttaggtcttggttctttcctaggggctggtttgtgggcagtggctttgttgcggcctcttggtgggtcatgaagctccacactttctttttctttgggagtgctgctggtaatatttggtttgggccaggtaaactcgtcagtgctggtgttcttctcaacttttttgggctgttttttcccaattgtcctttgagacactgtctcactagttgttgacaacttatgcttcaaagcctttgtttctggaattttctgagtgggccgtggacgggctttctccctaatgagactgaggagaggcctttctttgggttcagctgggacctgactggcattcgtcttcactttcatctggacttccattggttggatgattggaggaggcagagaaatagtctccatgggtgtttcattttggccacaaataaaagacttgttctgggatgtcactttgttaagccatttatccagttgccacttgttggttgagggtggctcaggctctggagttgccacacgaggtgcctcattagattcgctgtcagtggtgctactttcagtgtctgaatccgactcagagctgctctccgattcgctggagctgccagaacccccgctggcttgcactgcaggtgggggctggggagtggccaagggtgggttcacaggattattcctaggttttgccttttcaacagcctggtagagctcagtggcagtgcactgagtggtcaaggtcttcacaggctcaaggtcatcttcatcactgctcagcttcaggtcatcctcaagcatcgatttgaaagacactgactttgtagaagctctggtggttgggtcattccacttttgtaaggtgaatcctggggtcagatgctgcgattcccgcaagatttcttcaacacagcttggatcactgggaaggcttaccttcatcttgaagaaggacggaaatgcttggtgcctccttttgaacttcatggatcaagaaagaggggtgaagcatatcttacatctgggatagatagatgggccactgcaaccttcctctgggttgccacaaccaaaact

SEQ ID NO: 18739 - RNA, 10402 nt, Homo sapiens
  source 1..10402: mol_type = other RNA
tgagtgtgtgtgtgtgagtgtgtgtgtgtgtgtatttaatgaaagcctcattatatactttagtttatgccttcttgttactgagcttagttttcttcgtactgggtggaaaaagaattattttggtttggattattgtttctgaatagtcatgcaattgatacagagatattctggtttgagttcagagctaaaacagtaagtagatacttttaactaaaaacaaatgttaacaaaaaacttagattccctaataactaaagtaaaattcttatgaacaacaatgtgaaggtgggagaattactgagtttccacgtcacataaaagaaaaacacagtaaattctggattgtgctattctccatagagttcccgtaaatactttatcctagttacatgtaaaagttacaaatagcatttgtaaatcaaaataatgatgacaataataataaaataaaaaacactcacttatctttttaaaaaatcaatcgtgagggttttctgagtgcccattttacctgtgagatatggaaggagatgatggaaccatctccattgatccatctctcctttcagctcaggagggcttcattcttctcagctattctcctgcttaaaacctaggcttccagggcaacccatacctctagggccttatcataagctttctacattcacacattgattcatatcttaaaactatgtaattgttttagtcatcgaagtgtgtgtgtaagggtgagtttgtgtgtgtgtgtctgtgtgtgtccacatgaacacatatattaaatatgaaccctctgactggctgcatccagtggcgtgttgaagcatttttgcccaggcttgcaagagccaactgcgtgcatctctttccaaccatgtgttcagtgacatcacagttggtagcttaaaatcatctaaagtggtagtatttatgccatggaaattggcaaatggtgcaaaccaggtgctttctattctcagcgagctggttgttaaacattttaccagcacaccactggttgcatgctaggctgaccaaatgagaagctagatcttgttctgggcaacacggcattaacttagcctcgttggagtgtctccaattttgcttactgtccagggtctccttcctcccaatttcataaacactgcagaaccacaacagggcttgagcatctggggtgcatttgactacccattgtcaccacattgggctctattctcagagacactttcgtagccacatgagtgatgcaggacaaaaccaaaaaggtaaagcatctgaaattccctccgaatatgacagctggcttcctgctgcagagactggagaacaatgagttccccaataggaacaaactattcccagctgaaagcatcagctggggcattcttcaggaggcttcccacagctggtctgcatgctgctgctcaccagcaactgctggcaggcaggcgagcttgagcttgctactgcagcatcctgtcaggggcctggacgtaggcttccttcacttcccccttccctcctcaaagtctgatacaaatcacagagccaacaaaattgaggtcactggcaaaagagtttgaaattttgaatgatttttattaaacaccattagtctacactgcacagttaatgaaacagcaaagctccaatctcttagaagaatgatgactgatcatggatctaaaaagcagttcagtgtcccctaacccaatgtgagcactatgaataattctttaacatctcatgtcagacgcaaaaaggggcaagaactgcaatctggctttgtggggcttccccaccccccacccccccgcccccacccccaccccctttctgccctccccacaatgcaattttcttttagctggtagattacagagtaaaatgtgatgattttggtaaagagggcttctatatttctgaggaggaggatggaaagagaattaatactttttccttcaccaaaaatatcagatggtaggattaatgtctgagaccggcctatctgattagtctcctgccagggtaaatgctgattatgaatacacagatgccacttctgttgttggagtctactaacactaaagagaaaatgaattagattttaattatgagaataaggccgtgcgagtgaaaatgagaaacaacaacaacaataacaacaacgatgaagaatttagtctgccagtcatgtaacagaacactgacaactggctcaataatttttccccacagaattaaatttgggggtgctgaattgacccattcatttgatactgtgtagctgtatcatcttgccacacatttttctcaatggggatagtgatgcttctctaagcaagcagttcattgctttactgagtagtcttacccagtgatccagtttggttctcccacctgccaactcatgcaggtgaattttatcatgtctgttgagaagtatgtgaggcttcaccctcacaactcaactgattctgccttcaaagatattttccaacctcaaactccaacttcaacctccgggatgcaaatttgcatgaaacagaatccaaattagatatctttgggaaagatatgctagaagagtatctttccaatgcagacaaaatctaatgaatttagtgatgtaatgtccaaatgaaaattcatccatttggaaactcaacaaaacacatttttagccaatggtttctaattttgcaacttgctttttgcctgaagattttggtcttttcatttccttacatggaaaaaaaggcatcccgaccttaagtcttttaaaagtagtagcagctaatctgcttttccaattatgtcatccaaatataaaactactagtattttcccaatgagattattaagtaattaacagtctacaggctggctaacaacatgcttacagctaaattctacccggaggaccacactagtaaacccttttcaaagtaatcctacctaccaaactcagacagttatatgacaaaaccactaaaaatccaaagttaattaaaaatacaaagccaagccaacatcataacacaaacttgtcaaactctctgtggttggagcttgggtgacaagtgaaggcgtagtggtggccctacctgggtcaagttgcagggctgagatcatttggtgtacttgctcagatggagcttccttttactctgccctctattctaacctccacgtgcttatttaagtgtgtctcaccaagcctccatcaagatctagaggcacgatctctcactgccatccacatgtctcatatccctcccacaaactggtatactgaagagattcatttgacagaatatctccatcccttagtccctcaaatagctgcacacctacgacacgcatcaccatttacactgtgatgaacagagtaactataaaacagcaacaatccttaatcatgaaactgaaagatgtcttatctcaagggataggaaggtaattcatcctccatgtttaattagttcctaagctgctttataaatgagtctactacataatcaagtggtgatccagagctcgattgtcagatttggtcactgtgctgcagacttggcacatattttacactcagtcaccagagatgacagagaatcctcttgcctccctgttgtatgtaagtagatataacaagtcactgaaactagaactacaagtctttcatccatgaggcaatatgcttgtttctctgggaaactgcctcaacattctaatgtctagtttctggatgtgggatttcaagaagaatctactcctaaatccatgatggtctaggattgtggtttaggttgaacttacaagtcaagccagtgggcttcattatatagtaatagccaggcactctacctggtaaaccatgataaagagacaacttgagtcactgcaaagtcatcagcttaatttttatatgtgacaccaaccttgggtgttcagagtctttaatgttatcatcattttcctcttttaagaggctcagaaaagattctttcaggtttcatttgtgagtgtttggatgcataagtgttgttgctgagactgtaaacataaagctcaaccacagtgggagcataaaaagtgctgggttcagctgcagggatgctcccatcagccatattaacaacatggcttcagccattggagtacaacttccacagccttatacaacaaaaggccttaaactcaaagatgaccagagcacagctcaagtctggctgttttgcaactggggatatatctaaccttgacaatgagagtgcagagtcatcacctgctgtttctatcatggacctgcatggctggctttaataatcacacaagtttgcatctttcatgtgcatatctattatttatctggtcataactcagtgaacagaatttgataacccagcatattaaaggctacatggaattatataccagcaggtaattaccagtaagtaatgcatggatagtgtttaccccaagtgtaagaatcttctggtgagctggaacatcaaaaatgatatttacattgtgatgtttagggacataaaatgaatgtgaaggatcataagggggtagtcacaaccagtgagaaatgtctccaaattaggtgaatggttcccaatgtttagggctctttcaaagcatctcaaggtgaagcactaccccacgactcattttaaaaaaataaaagttagctactatttagagagtttggagttttcttagaaattttcatggaaatgattcacaataatatggactttaataaaaggagtaattgtaattcagtcaaaagttaatgagccaaacaaaggaaagggaaacacagataagagaaaaaagaaagtagaaaacagaaaacctataagagagaaaatgtgaataataattgaggaagtccagattttcaagccactaggaagaaaactgtatatcattacttctaggtagtgataccttgacttttgttcccatagatttgagcaaaatacaatttaaaaatcctgccagttatggacccacttaccaactgtgtaaatgttgttgttgcaaaggaggcagaggtgtgaattccttgttggacactttccagacctctcttaactcccacttgtaagtctagagtgtagcattttggctactaaggcatgcatcaaccaaactgttcttcaaaaggacagctttgcacacagagaaccccaggtgaggatttacacttcaaataatggagttgaaaaacactgatgccagctgatgcctaaaacttgtcaaaataaatgtcaccctttcttcttatcattaaaattaacaaaatagggaatcaggaaagggatgctaacaagaaagtcctctggttgtgtggcatagcatctttttaagagtagcattgctatgctcatttattttcttgatactcttgattttatgatgttgctacaacatctaaccagtgggttttgacaatgaaaattctcacctgaagattgaatctgtgggatacacaaaagtttgacagattctgaaatatgttcttttctgggtataagagtagagtttgggggatggtcccttgtgtctaagttctcatgtatatgtaagaccacttgttgcatttctcaggagcctgtctttatcacaagtgcttcccattctttgttttgggtagtgtgggcttaaaacaatattgtagggactgtcattccataaagcacaaaaagatggtggaatctgagaaatgcatatcaaatgctaaaagaaaaaaaatgactaagtaataaaacgtacactgcccttaagttgtagtgtcaacttacaatgacttctgttttttacagataacaaaagaagcataaaaacaaacataaccaaagagaacgttccccagtgagtggagttccaccagtgaccatcagtgcgctggtagaggtagagtgatgggtcgtgatgctagagatctgagaacacccactacaacaagtgggcatcgatgcgcagccaacacagtccttggcgaacgtagcggacaagattggtcatgctgctgtgctgggtcagaggccccatcagcgtgtccagatcaccaaagaattctttgttttctcttgtcagtttgtcggccatatcccagtgttcatagccccgtaacacattgctagtgatgttgacgtggctggcagccatgtggtgaatgcgctggggaatggtgactgggccattgttacagttccccattgcgttgatgggggagacgttgttgagagacactggggatggagtgttctttccattgcttacccatggagagggtatctgtgcgacttttgaagcattttgcttaaaatattccatcagtgatctggagtacttcatagcatggtccttcttcagcttaaacattctcaaatagaggagtgataaacatcggtagcatagtactgctagctttttgtccccatccgaagccaagggacttgcaaagttcttcagcctcattgcatacctgaggagctccacagtctcagagtacatggtgtatggggactttgcttccagagggtcgcgttccatggcattgccacattcagtgaaggagagggcggcatcagcataattcacagctttgccaaatttctcgaacagtgcatcagctttgtgcttcagcttcttagcttcttgcatgtaataatcagcattgtgaaccgagtcatcaaaagtgagcttgggtctccggacattagtgctgctgctggatagaaggggcagagccgcccaggacgtcatctccaggtgactgctatccatgaggccagtagtgatggtagaggtgatggtggaaatggtagtggtagtagttgtggtggtggccgtggcggtggcagtagctgtgacagtggtggtgacaatggcagtagcagtgacagtagcagtggcaatagcagtattggtgacagtgatggtggcagaggatgccttttttggagtgtctccctcatttaccgatatccctttgaaagtagcacagaatttgccttcagttctcttaggtttggtagatgtgatttgtccagtcatggcgatgtttttgtcttgaccaaagggaccattattgccactgacatttctgcggcgtggagggtcctctggcagtggggaaagtggaggaggaaatagtttttcttcctttcttctatttgctctcctggatgaattattttctctagtgttgggaggcttgtggggtggggctggtgagatgcaaggagggagcaagcagatagttgtggcctcctccaggcgctgcttcttctcagggatcttctctgcaacttctattggcttgtgcttacgtttgcccttaggggctggtttctccacagctgtgacagctgtctgacgcttgggttttgtggcagtctccttgtggtctggcttggcaggtgctgcatggagtgagctgtggccaggtactctagagagtaagtcaaggtcaatcttcacccagaggtttttcaggttctcatgatctcgcagaggggacaggatttcagtttgcatgacaggaataggtgaaaatgttggctcttcattactgatggataagttgttgttgctgccactgctactcattaaggtgctgagggtcaggctggcaccacagatttccttggatttggcagtattacctccagaaataatgcacggaggcaggactttgatttgcagggtctcttcctgatctgtgttggagtcagatgtagatgaatctgtttcaatgaattcccgagactttggcacaatcttgccaggccctctgtacttcttcttctcgggagccaaagggatgttaggtcttggttctttcctaggggctggtttgtgggcagtggctttgttgcggcctcttggtgggtcatgaagctccacactttctttttctttgggagtgctgctggtaatatttggtttgggccaggtaaactcgtcagtgctggtgttcttctcaacttttttgggctgttttttcccaattgtcctttgagacactgtctcactagttgttgacaacttatgcttcaaagcctttgtttctggaattttctgagtgggccgtggacgggctttctccctaatgagactgaggagaggcctttctttgggttcagctgggacctgactggcattcgtcttcactttcatctggacttccattggttggatgattggaggaggcagagaaatagtctccatgggtgtttcattttggccacaaataaaagacttgttctgggatgtcactttgttaagccatttatccagttgccacttgttggttgagggtggctcaggctctggagttgccacacgaggtgcctcattagattcgctgtcagtggtgctactttcagtgtctgaatccgactcagagctgctctccgattcgctggagctgccagaacccccgctggcttgcactgcaggtgggggctggggagtggccaagggtgggttcacaggattattcctaggttttgccttttcaacagcctggtagagctcagtggcagtgcactgagtggtcaaggtcttcacaggctcaaggtcatcttcatcactgctcagcttcaggtcatcctcaagcatcgatttgaaagacactgactttgtagaagctctggtggttgggtcattccacttttgtaaggtgaatcctggggtcagatgctgcgattcctgtcctgggatggaaaaggtgctctgctcagagtgtccagcagtatgcatggaagtgagaggagtaggccaggaatgggtcatctcccgcaagatttcttcaacacagcttggatcactgggaaggcttacttcacttgtttggaggatggtgaactttggcagtttagtctttgaactggctgcactgggttttccatccaagagtgttccaaatgacagattcccaaagctgttctcaaattcaattgaaggtttcagtgttggtgagatgtccggtgcctggtcctggccatccatgggtctgacgtatgcagttggcttttgctgccccatgcttgttttgcagtaaagccctggtgggaagttttgaactgaaaggccactgctaggagctaataaagaggaagccactaggggagacccaggcgcttgcacggcgaattcagattcttccggtgaattggattgaaagatttctttgaaagcatcttctccactagaattagggttactgtcttcctttgcagatgggtttgactcttcaacttctccaatctggggctgttcagctgggtagacaaagaagtcttccagtttggcttgagactggtcctgtgtcaaagtctgcatcttgtttggctgaccactggcctggcttgccagtacagtgctagggttatgactatcacgtgaccactcaggttttgattttctgttgctgtgtattagagttgaattcagtatcacaacagaaggtggaggcattggtgctgaaggatgggtattatcctggtgaggtggaattattctgttcttttgttctggaaaaaagcttggttcatttttgttgttgggattctggggcacagaattctttggaattcccactaggtgattctgattagaatggttagttagcaaattcttcatttcatcatagtttccaagcgtgttctggactcggttggcaagtgcatcacctttgtttgtatattcagctaccttgtatggctccccaaaaagatcaaagcctgaagaaaagagatcgtcttcttgctggacttcttgattcctccgctcccattccctttttttaagtgcactacggtcttgttcatagtgacactgctgctccaagtcccagtctctgaaaaagtcgaatagatccatagcggccaggcggcggcggcgggcgggcgcctgtccctgatcgcagcgggtcggcgcggctctcggcacagctcgctggcggttctcggcggcccccggctctccagccctcccgcccagctaaaagtgtccgggccgcatcggcagcagcagcgggcgctggaggtgtctggtcctgtgctccggcgaggaagcggcggcagtggcactgggcgggcaagcgcctggtcgcccactcgggtccgctcggtccgcggtagcccgcgcacccagcgacccgacgctgcggcggcagccgctgcgggctcaggcgggctgggccgcccgcctggctggctgcgggccggcggcggcagcggcggcgggggcggccggggcagaggcagcggcgcggcgcggcagccggggcggcagcggcggcggcggcggcggcggcggcggcggcggcggcggcggcggcagcggctgcacaggcggcggc

SEQ ID NO: 18740 - RNA, 10297 nt, Homo sapiens
  source 1..10297: mol_type = other RNA
tgagtgtgtgtgtgtgagtgtgtgtgtgtgtgtatttaatgaaagcctcattatatactttagtttatgccttcttgttactgagcttagttttcttcgtactgggtggaaaaagaattattttggtttggattattgtttctgaatagtcatgcaattgatacagagatattctggtttgagttcagagctaaaacagtaagtagatacttttaactaaaaacaaatgttaacaaaaaacttagattccctaataactaaagtaaaattcttatgaacaacaatgtgaaggtgggagaattactgagtttccacgtcacataaaagaaaaacacagtaaattctggattgtgctattctccatagagttcccgtaaatactttatcctagttacatgtaaaagttacaaatagcatttgtaaatcaaaataatgatgacaataataataaaataaaaaacactcacttatctttttaaaaaatcaatcgtgagggttttctgagtgcccattttacctgtgagatatggaaggagatgatggaaccatctccattgatccatctctcctttcagctcaggagggcttcattcttctcagctattctcctgcttaaaacctaggcttccagggcaacccatacctctagggccttatcataagctttctacattcacacattgattcatatcttaaaactatgtaattgttttagtcatcgaagtgtgtgtgtaagggtgagtttgtgtgtgtgtgtctgtgtgtgtccacatgaacacatatattaaatatgaaccctctgactggctgcatccagtggcgtgttgaagcatttttgcccaggcttgcaagagccaactgcgtgcatctctttccaaccatgtgttcagtgacatcacagttggtagcttaaaatcatctaaagtggtagtatttatgccatggaaattggcaaatggtgcaaaccaggtgctttctattctcagcgagctggttgttaaacattttaccagcacaccactggttgcatgctaggctgaccaaatgagaagctagatcttgttctgggcaacacggcattaacttagcctcgttggagtgtctccaattttgcttactgtccagggtctccttcctcccaatttcataaacactgcagaaccacaacagggcttgagcatctggggtgcatttgactacccattgtcaccacattgggctctattctcagagacactttcgtagccacatgagtgatgcaggacaaaaccaaaaaggtaaagcatctgaaattccctccgaatatgacagctggcttcctgctgcagagactggagaacaatgagttccccaataggaacaaactattcccagctgaaagcatcagctggggcattcttcaggaggcttcccacagctggtctgcatgctgctgctcaccagcaactgctggcaggcaggcgagcttgagcttgctactgcagcatcctgtcaggggcctggacgtaggcttccttcacttcccccttccctcctcaaagtctgatacaaatcacagagccaacaaaattgaggtcactggcaaaagagtttgaaattttgaatgatttttattaaacaccattagtctacactgcacagttaatgaaacagcaaagctccaatctcttagaagaatgatgactgatcatggatctaaaaagcagttcagtgtcccctaacccaatgtgagcactatgaataattctttaacatctcatgtcagacgcaaaaaggggcaagaactgcaatctggctttgtggggcttccccaccccccacccccccgcccccacccccaccccctttctgccctccccacaatgcaattttcttttagctggtagattacagagtaaaatgtgatgattttggtaaagagggcttctatatttctgaggaggaggatggaaagagaattaatactttttccttcaccaaaaatatcagatggtaggattaatgtctgagaccggcctatctgattagtctcctgccagggtaaatgctgattatgaatacacagatgccacttctgttgttggagtctactaacactaaagagaaaatgaattagattttaattatgagaataaggccgtgcgagtgaaaatgagaaacaacaacaacaataacaacaacgatgaagaatttagtctgccagtcatgtaacagaacactgacaactggctcaataatttttccccacagaattaaatttgggggtgctgaattgacccattcatttgatactgtgtagctgtatcatcttgccacacatttttctcaatggggatagtgatgcttctctaagcaagcagttcattgctttactgagtagtcttacccagtgatccagtttggttctcccacctgccaactcatgcaggtgaattttatcatgtctgttgagaagtatgtgaggcttcaccctcacaactcaactgattctgccttcaaagatattttccaacctcaaactccaacttcaacctccgggatgcaaatttgcatgaaacagaatccaaattagatatctttgggaaagatatgctagaagagtatctttccaatgcagacaaaatctaatgaatttagtgatgtaatgtccaaatgaaaattcatccatttggaaactcaacaaaacacatttttagccaatggtttctaattttgcaacttgctttttgcctgaagattttggtcttttcatttccttacatggaaaaaaaggcatcccgaccttaagtcttttaaaagtagtagcagctaatctgcttttccaattatgtcatccaaatataaaactactagtattttcccaatgagattattaagtaattaacagtctacaggctggctaacaacatgcttacagctaaattctacccggaggaccacactagtaaacccttttcaaagtaatcctacctaccaaactcagacagttatatgacaaaaccactaaaaatccaaagttaattaaaaatacaaagccaagccaacatcataacacaaacttgtcaaactctctgtggttggagcttgggtgacaagtgaaggcgtagtggtggccctacctgggtcaagttgcagggctgagatcatttggtgtacttgctcagatggagcttccttttactctgccctctattctaacctccacgtgcttatttaagtgtgtctcaccaagcctccatcaagatctagaggcacgatctctcactgccatccacatgtctcatatccctcccacaaactggtatactgaagagattcatttgacagaatatctccatcccttagtccctcaaatagctgcacacctacgacacgcatcaccatttacactgtgatgaacagagtaactataaaacagcaacaatccttaatcatgaaactgaaagatgtcttatctcaagggataggaaggtaattcatcctccatgtttaattagttcctaagctgctttataaatgagtctactacataatcaagtggtgatccagagctcgattgtcagatttggtcactgtgctgcagacttggcacatattttacactcagtcaccagagatgacagagaatcctcttgcctccctgttgtatgtaagtagatataacaagtcactgaaactagaactacaagtctttcatccatgaggcaatatgcttgtttctctgggaaactgcctcaacattctaatgtctagtttctggatgtgggatttcaagaagaatctactcctaaatccatgatggtctaggattgtggtttaggttgaacttacaagtcaagccagtgggcttcattatatagtaatagccaggcactctacctggtaaaccatgataaagagacaacttgagtcactgcaaagtcatcagcttaatttttatatgtgacaccaaccttgggtgttcagagtctttaatgttatcatcattttcctcttttaagaggctcagaaaagattctttcaggtttcatttgtgagtgtttggatgcataagtgttgttgctgagactgtaaacataaagctcaaccacagtgggagcataaaaagtgctgggttcagctgcagggatgctcccatcagccatattaacaacatggcttcagccattggagtacaacttccacagccttatacaacaaaaggccttaaactcaaagatgaccagagcacagctcaagtctggctgttttgcaactggggatatatctaaccttgacaatgagagtgcagagtcatcacctgctgtttctatcatggacctgcatggctggctttaataatcacacaagtttgcatctttcatgtgcatatctattatttatctggtcataactcagtgaacagaatttgataacccagcatattaaaggctacatggaattatataccagcaggtaattaccagtaagtaatgcatggatagtgtttaccccaagtgtaagaatcttctggtgagctggaacatcaaaaatgatatttacattgtgatgtttagggacataaaatgaatgtgaaggatcataagggggtagtcacaaccagtgagaaatgtctccaaattaggtgaatggttcccaatgtttagggctctttcaaagcatctcaaggtgaagcactaccccacgactcattttaaaaaaataaaagttagctactatttagagagtttggagttttcttagaaattttcatggaaatgattcacaataatatggactttaataaaaggagtaattgtaattcagtcaaaagttaatgagccaaacaaaggaaagggaaacacagataagagaaaaaagaaagtagaaaacagaaaacctataagagagaaaatgtgaataataattgaggaagtccagattttcaagccactaggaagaaaactgtatatcattacttctaggtagtgataccttgacttttgttcccatagatttgagcaaaatacaatttaaaaatcctgccagttatggacccacttaccaactgtgtaaatgttgttgttgcaaaggaggcagaggtgtgaattccttgttggacactttccagacctctcttaactcccacttgtaagtctagagtgtagcattttggctactaaggcatgcatcaaccaaactgttcttcaaaaggacagctttgcacacagagaaccccaggtgaggatttacacttcaaataatggagttgaaaaacactgatgccagctgatgcctaaaacttgtcaaaataaatgtcaccctttcttcttatcattaaaattaacaaaatagggaatcaggaaagggatgctaacaagaaagtcctctggttgtgtggcatagcatctttttaagagtagcattgctatgctcatttattttcttgatactcttgattttatgatgttgctacaacatctaaccagtgggttttgacaatgaaaattctcacctgaagattgaatctgtgggatacacaaaagtttgacagattctgaaatatgttcttttctgggtataagagtagagtttgggggatggtcccttgtgtctaagttctcatgtatatgtaagaccacttgttgcatttctcaggagcctgtctttatcacaagtgcttcccattctttgttttgggtagtgtgggcttaaaacaatattgtagggactgtcattccataaagcacaaaaagatggtggaatctgagaaatgcatatcaaatgctaaaagaaaaaaaatgactaagtaataaaacgtacactgcccttaagttgtagtgtcaacttacaatgacttctgttttttacagataacaaaagaagcataaaaacaaacataaccaaagagaacgttccccagtgagtggagttccaccagtgaccatcagtgcgctggtagaggtagagtgatgggtcgtgatgctagagatctgagaacacccactacaacaagtgggcatcgatgcgcagccaacacagtccttggcgaacgtagcggacaagattggtcatgctgctgtgctgggtcagaggccccatcagcgtgtccagatcaccaaagaattctttgttttctcttgtcagtttgtcggccatatcccagtgttcatagccccgtaacacattgctagtgatgttgacgtggctggcagccatgtggtgaatgcgctggggaatggtgactgggccattgttacagttccccattgcgttgatgggggagacgttgttgagagacactggggatggagtgttctttccattgcttacccatggagagggtatctgtgcgacttttgaagcattttgcttaaaatattccatcagtgatctggagtacttcatagcatggtccttcttcagcttaaacattctcaaatagaggagtgataaacatcggtagcatagtactgctagctttttgtccccatccgaagccaagggacttgcaaagttcttcagcctcattgcatacctgaggagctccacagtctcagagtacatggtgtatggggactttgcttccagagggtcgcgttccatggcattgccacattcagtgaaggagagggcggcatcagcataattcacagctttgccaaatttctcgaacagtgcatcagctttgtgcttcagcttcttagcttcttgcatgtaataatcagcattgtgaaccgagtcatcaaaagtgagcttgggtctccggacattagtgctgctgctggatagaaggggcagagccgcccaggacgtcatctccaggtgactgctatccatgaggccagtagtgatggtagaggtgatggtggaaatggtagtggtagtagttgtggtggtggccgtggcggtggcagtagctgtgacagtggtggtgacaatggcagtagcagtgacagtagcagtggcaatagcagtattggtgacagtgatggtggcagaggatgccttttttggagtgtctccctcatttaccgatatccctttgaaagtagcacagaatttgccttcagttctcttaggtttggtagatgtgatttgtccagtcatggcgatgtttttgtcttgaccaaagggaccattattgccactgacatttctgcggcgtggagggtcctctggcagtggggaaagtggaggaggaaatagtttttcttcctttcttctatttgctctcctggatgaattattttctctagtgttgggaggcttgtggggtggggctggtgagatgcaaggagggagcaagcagatagttgtggcctcctccaggcgctgcttcttctcagggatcttctctgcaacttctattggcttgtgcttacgtttgcccttaggggctggtttctccacagctgtgacagctgtctgacgcttgggttttgtggcagtctccttgtggtctggcttggcaggtgctgcatggagtgagctgtggccaggtactctagagagtaagtcaaggtcaatcttcacccagaggtttttcaggttctcatgatctcgcagaggggacaggatttcagtttgcatgacaggaataggtgaaaatgttggctcttcattactgatggataagttgttgttgctgccactgctactcattaaggtgctgagggtcaggctggcaccacagatttccttggatttggcagtattacctccagaaataatgcacggaggcaggactttgatttgcagggtctcttcctgatctgtgttggagtcagatgtagatgaatctgtttcaatgaattcccgagactttggcacaatcttgccaggccctctgtacttcttcttctcgggagccaaagggatgttaggtcttggttctttcctaggggctggtttgtgggcagtggctttgttgcggcctcttggtgggtcatgaagctccacactttctttttctttgggagtgctgctggtaatatttggtttgggccaggtaaactcgtcagtgctggtgttcttctcaacttttttgggctgttttttcccaattgtcctttgagacactgtctcactagttgttgacaacttatgcttcaaagcctttgtttctggaattttctgagtgggccgtggacgggctttctccctaatgagactgaggagaggcctttctttgggttcagctgggacctgactggcattcgtcttcactttcatctggacttccattggttggatgattggaggaggcagagaaatagtctccatgggtgtttcattttggccacaaataaaagacttgttctgggatgtcactttgttaagccatttatccagttgccacttgttggttgagggtggctcaggctctggagttgccacacgaggtgcctcattagattcgctgtcagtggtgctactttcagtgtctgaatccgactcagagctgctctccgattcgctggagctgccagaacccccgctggcttgcactgcaggtgggggctggggagtggccaagggtgggttcacaggattattcctaggttttgccttttcaacagcctggtagagctcagtggcagtgcactgagtggtcaaggtcttcacaggctcaaggtcatcttcatcactgctcagcttcaggtcatcctcaagcatctttgtagaagctctggtggttgggtcattccacttttgtaaggtgaatcctggggtcagatgctgcgattcccgcaagatttcttcaacacagcttggatcactgggaaggcttacttcacttgtttggaggatggtgaactttggcagtttagtctttgaactggctgcactgggttttccatccaagagtgttccaaatgacagattcccaaagctgttctcaaattcaattgaaggtttcagtgttggtgagatgtccggtgcctggtcctggccatccatgggtctgacgtatgcagttggcttttgctgccccatgcttgttttgcagtaaagccctggtgggaagttttgaactgaaaggccactgctaggagctaataaagaggaagccactaggggagacccaggcgcttgcacggcgaattcagattcttccggtgaattggattgaaagatttctttgaaagcatcttctccactagaattagggttactgtcttcctttgcagatgggtttgactcttcaacttctccaatctggggctgttcagctgggtagacaaagaagtcttccagtttggcttgagactggtcctgtgtcaaagtctgcatcttgtttggctgaccactggcctggcttgccagtacagtgctagggttatgactatcacgtgaccactcaggttttgattttctgttgctgtgtattagagttgaattcagtatcacaacagaaggtggaggcattggtgctgaaggatgggtattatcctggtgaggtggaattattctgttcttttgttctggaaaaaagcttggttcatttttgttgttgggattctggggcacagaattctttggaattcccactaggtgattctgattagaatggttagttagcaaattcttcatttcatcatagtttccaagcgtgttctggactcggttggcaagtgcatcacctttgtttgtatattcagctaccttgtatggctccccaaaaagatcaaagcctgaagaaaagagatcgtcttcttgctggacttcttgattcctccgctcccattccctttttttaagtgcactacggtcttgttcatagtgacactgctgctccaagtcccagtctctgaaaaagtcgaatagatccatagcggccaggcggcggcggcgggcgggcgcctgtccctgatcgcagcgggtcggcgcggctctcggcacagctcgctggcggttctcggcggcccccggctctccagccctcccgcccagctaaaagtgtccgggccgcatcggcagcagcagcgggcgctggaggtgtctggtcctgtgctccggcgaggaagcggcggcagtggcactgggcgggcaagcgcctggtcgcccactcgggtccgctcggtccgcggtagcccgcgcacccagcgacccgacgctgcggcggcagccgctgcgggctcaggcgggctgggccgcccgcctggctggctgcgggccggcggcggcagcggcggcgggggcggccggggcagaggcagcggcgcggcgcggcagccggggcggcagcggcggcggcggcggcggcggcggcggcggcggcggcggcggcggcagcggctgcacaggcggcggc

SEQ ID NO: 18741 - RNA, 10285 nt, Homo sapiens
  source 1..10285: mol_type = other RNA
tgagtgtgtgtgtgtgagtgtgtgtgtgtgtgtatttaatgaaagcctcattatatactttagtttatgccttcttgttactgagcttagttttcttcgtactgggtggaaaaagaattattttggtttggattattgtttctgaatagtcatgcaattgatacagagatattctggtttgagttcagagctaaaacagtaagtagatacttttaactaaaaacaaatgttaacaaaaaacttagattccctaataactaaagtaaaattcttatgaacaacaatgtgaaggtgggagaattactgagtttccacgtcacataaaagaaaaacacagtaaattctggattgtgctattctccatagagttcccgtaaatactttatcctagttacatgtaaaagttacaaatagcatttgtaaatcaaaataatgatgacaataataataaaataaaaaacactcacttatctttttaaaaaatcaatcgtgagggttttctgagtgcccattttacctgtgagatatggaaggagatgatggaaccatctccattgatccatctctcctttcagctcaggagggcttcattcttctcagctattctcctgcttaaaacctaggcttccagggcaacccatacctctagggccttatcataagctttctacattcacacattgattcatatcttaaaactatgtaattgttttagtcatcgaagtgtgtgtgtaagggtgagtttgtgtgtgtgtgtctgtgtgtgtccacatgaacacatatattaaatatgaaccctctgactggctgcatccagtggcgtgttgaagcatttttgcccaggcttgcaagagccaactgcgtgcatctctttccaaccatgtgttcagtgacatcacagttggtagcttaaaatcatctaaagtggtagtatttatgccatggaaattggcaaatggtgcaaaccaggtgctttctattctcagcgagctggttgttaaacattttaccagcacaccactggttgcatgctaggctgaccaaatgagaagctagatcttgttctgggcaacacggcattaacttagcctcgttggagtgtctccaattttgcttactgtccagggtctccttcctcccaatttcataaacactgcagaaccacaacagggcttgagcatctggggtgcatttgactacccattgtcaccacattgggctctattctcagagacactttcgtagccacatgagtgatgcaggacaaaaccaaaaaggtaaagcatctgaaattccctccgaatatgacagctggcttcctgctgcagagactggagaacaatgagttccccaataggaacaaactattcccagctgaaagcatcagctggggcattcttcaggaggcttcccacagctggtctgcatgctgctgctcaccagcaactgctggcaggcaggcgagcttgagcttgctactgcagcatcctgtcaggggcctggacgtaggcttccttcacttcccccttccctcctcaaagtctgatacaaatcacagagccaacaaaattgaggtcactggcaaaagagtttgaaattttgaatgatttttattaaacaccattagtctacactgcacagttaatgaaacagcaaagctccaatctcttagaagaatgatgactgatcatggatctaaaaagcagttcagtgtcccctaacccaatgtgagcactatgaataattctttaacatctcatgtcagacgcaaaaaggggcaagaactgcaatctggctttgtggggcttccccaccccccacccccccgcccccacccccaccccctttctgccctccccacaatgcaattttcttttagctggtagattacagagtaaaatgtgatgattttggtaaagagggcttctatatttctgaggaggaggatggaaagagaattaatactttttccttcaccaaaaatatcagatggtaggattaatgtctgagaccggcctatctgattagtctcctgccagggtaaatgctgattatgaatacacagatgccacttctgttgttggagtctactaacactaaagagaaaatgaattagattttaattatgagaataaggccgtgcgagtgaaaatgagaaacaacaacaacaataacaacaacgatgaagaatttagtctgccagtcatgtaacagaacactgacaactggctcaataatttttccccacagaattaaatttgggggtgctgaattgacccattcatttgatactgtgtagctgtatcatcttgccacacatttttctcaatggggatagtgatgcttctctaagcaagcagttcattgctttactgagtagtcttacccagtgatccagtttggttctcccacctgccaactcatgcaggtgaattttatcatgtctgttgagaagtatgtgaggcttcaccctcacaactcaactgattctgccttcaaagatattttccaacctcaaactccaacttcaacctccgggatgcaaatttgcatgaaacagaatccaaattagatatctttgggaaagatatgctagaagagtatctttccaatgcagacaaaatctaatgaatttagtgatgtaatgtccaaatgaaaattcatccatttggaaactcaacaaaacacatttttagccaatggtttctaattttgcaacttgctttttgcctgaagattttggtcttttcatttccttacatggaaaaaaaggcatcccgaccttaagtcttttaaaagtagtagcagctaatctgcttttccaattatgtcatccaaatataaaactactagtattttcccaatgagattattaagtaattaacagtctacaggctggctaacaacatgcttacagctaaattctacccggaggaccacactagtaaacccttttcaaagtaatcctacctaccaaactcagacagttatatgacaaaaccactaaaaatccaaagttaattaaaaatacaaagccaagccaacatcataacacaaacttgtcaaactctctgtggttggagcttgggtgacaagtgaaggcgtagtggtggccctacctgggtcaagttgcagggctgagatcatttggtgtacttgctcagatggagcttccttttactctgccctctattctaacctccacgtgcttatttaagtgtgtctcaccaagcctccatcaagatctagaggcacgatctctcactgccatccacatgtctcatatccctcccacaaactggtatactgaagagattcatttgacagaatatctccatcccttagtccctcaaatagctgcacacctacgacacgcatcaccatttacactgtgatgaacagagtaactataaaacagcaacaatccttaatcatgaaactgaaagatgtcttatctcaagggataggaaggtaattcatcctccatgtttaattagttcctaagctgctttataaatgagtctactacataatcaagtggtgatccagagctcgattgtcagatttggtcactgtgctgcagacttggcacatattttacactcagtcaccagagatgacagagaatcctcttgcctccctgttgtatgtaagtagatataacaagtcactgaaactagaactacaagtctttcatccatgaggcaatatgcttgtttctctgggaaactgcctcaacattctaatgtctagtttctggatgtgggatttcaagaagaatctactcctaaatccatgatggtctaggattgtggtttaggttgaacttacaagtcaagccagtgggcttcattatatagtaatagccaggcactctacctggtaaaccatgataaagagacaacttgagtcactgcaaagtcatcagcttaatttttatatgtgacaccaaccttgggtgttcagagtctttaatgttatcatcattttcctcttttaagaggctcagaaaagattctttcaggtttcatttgtgagtgtttggatgcataagtgttgttgctgagactgtaaacataaagctcaaccacagtgggagcataaaaagtgctgggttcagctgcagggatgctcccatcagccatattaacaacatggcttcagccattggagtacaacttccacagccttatacaacaaaaggccttaaactcaaagatgaccagagcacagctcaagtctggctgttttgcaactggggatatatctaaccttgacaatgagagtgcagagtcatcacctgctgtttctatcatggacctgcatggctggctttaataatcacacaagtttgcatctttcatgtgcatatctattatttatctggtcataactcagtgaacagaatttgataacccagcatattaaaggctacatggaattatataccagcaggtaattaccagtaagtaatgcatggatagtgtttaccccaagtgtaagaatcttctggtgagctggaacatcaaaaatgatatttacattgtgatgtttagggacataaaatgaatgtgaaggatcataagggggtagtcacaaccagtgagaaatgtctccaaattaggtgaatggttcccaatgtttagggctctttcaaagcatctcaaggtgaagcactaccccacgactcattttaaaaaaataaaagttagctactatttagagagtttggagttttcttagaaattttcatggaaatgattcacaataatatggactttaataaaaggagtaattgtaattcagtcaaaagttaatgagccaaacaaaggaaagggaaacacagataagagaaaaaagaaagtagaaaacagaaaacctataagagagaaaatgtgaataataattgaggaagtccagattttcaagccactaggaagaaaactgtatatcattacttctaggtagtgataccttgacttttgttcccatagatttgagcaaaatacaatttaaaaatcctgccagttatggacccacttaccaactgtgtaaatgttgttgttgcaaaggaggcagaggtgtgaattccttgttggacactttccagacctctcttaactcccacttgtaagtctagagtgtagcattttggctactaaggcatgcatcaaccaaactgttcttcaaaaggacagctttgcacacagagaaccccaggtgaggatttacacttcaaataatggagttgaaaaacactgatgccagctgatgcctaaaacttgtcaaaataaatgtcaccctttcttcttatcattaaaattaacaaaatagggaatcaggaaagggatgctaacaagaaagtcctctggttgtgtggcatagcatctttttaagagtagcattgctatgctcatttattttcttgatactcttgattttatgatgttgctacaacatctaaccagtgggttttgacaatgaaaattctcacctgaagattgaatctgtgggatacacaaaagtttgacagattctgaaatatgttcttttctgggtataagagtagagtttgggggatggtcccttgtgtctaagttctcatgtatatgtaagaccacttgttgcatttctcaggagcctgtctttatcacaagtgcttcccattctttgttttgggtagtgtgggcttaaaacaatattgtagggactgtcattccataaagcacaaaaagatggtggaatctgagaaatgcatatcaaatgctaaaagaaaaaaaatgactaagtaataaaacgtacactgcccttaagttgtagtgtcaacttacaatgacttctgttttttacagataacaaaagaagcataaaaacaaacataaccaaagagaacgttccccagtgagtggagttccaccagtgaccatcagtgcgctggtagaggtagagtgatgggtcgtgatgctagagatctgagaacacccactacaacaagtgggcatcgatgcgcagccaacacagtccttggcgaacgtagcggacaagattggtcatgctgctgtgctgggtcagaggccccatcagcgtgtccagatcaccaaagaattctttgttttctcttgtcagtttgtcggccatatcccagtgttcatagccccgtaacacattgctagtgatgttgacgtggctggcagccatgtggtgaatgcgctggggaatggtgactgggccattgttacagttccccattgcgttgatgggggagacgttgttgagagacactggggatggagtgttctttccattgcttacccatggagagggtatctgtgcgacttttgaagcattttgcttaaaatattccatcagtgatctggagtacttcatagcatggtccttcttcagcttaaacattctcaaatagaggagtgataaacatcggtagcatagtactgctagctttttgtccccatccgaagccaagggacttgcaaagttcttcagcctcattgcatacctgaggagctccacagtctcagagtacatggtgtatggggactttgcttccagagggtcgcgttccatggcattgccacattcagtgaaggagagggcggcatcagcataattcacagctttgccaaatttctcgaacagtgcatcagctttgtgcttcagcttcttagcttcttgcatgtaataatcagcattgtgaaccgagtcatcaaaagtgagcttgggtctccggacattagtgctgctgctggatagaaggggcagagccgcccaggacgtcatctccaggtgactgctatccatgaggccagtagtgatggtagaggtgatggtggaaatggtagtggtagtagttgtggtggtggccgtggcggtggcagtagctgtgacagtggtggtgacaatggcagtagcagtgacagtagcagtggcaatagcagtattggtgacagtgatggtggcagaggatgccttttttggagtgtctccctcatttaccgatatccctttgaaagtagcacagaatttgccttcagttctcttaggtttggtagatgtgatttgtccagtcatggcgatgtttttgtcttgaccaaagggaccattattgccactgacatttctgcggcgtggagggtcctctggcagtggggaaagtggaggaggaaatagtttttcttcctttcttctatttgctctcctggatgaattattttctctagtgttgggaggcttgtggggtggggctggtgagatgcaaggagggagcaagcagatagttgtggcctcctccaggcgctgcttcttctcagggatcttctctgcaacttctattggcttgtgcttacgtttgcccttaggggctggtttctccacagctgtgacagctgtctgacgcttgggttttgtggcagtctccttgtggtctggcttggcaggtgctgcatggagtgagctgtggccaggtactctagagagtaagtcaaggtcaatcttcacccagaggtttttcaggttctcatgatctcgcagaggggacaggatttcagtttgcatgacaggaataggtgaaaatgttggctcttcattactgatggataagttgttgttgctgccactgctactcattaaggtgctgagggtcaggctggcaccacagatttccttggatttggcagtattacctccagaaataatgcacggaggcaggactttgatttgcagggtctcttcctgatctgtgttggagtcagatgtagatgaatctgtttcaatgaattcccgagactttggcacaatcttgccaggccctctgtacttcttcttctcgggagccaaagggatgttaggtcttggttctttcctaggggctggtttgtgggcagtggctttgttgcggcctcttggtgggtcatgaagctccacactttctttttctttgggagtgctgctggtaatatttggtttgggccaggtaaactcgtcagtgctggtgttcttctcaacttttttgggctgttttttcccaattgtcctttgagacactgtctcactagttgttgacaacttatgcttcaaagcctttgtttctggaattttctgagtgggccgtggacgggctttctccctaatgagactgaggagaggcctttctttgggttcagctgggacctgactggcattcgtcttcactttcatctggacttccattggttggatgattggaggaggcagagaaatagtctccatgggtgtttcattttggccacaaataaaagacttgttctgggatgtcactttgttaagccatttatccagttgccacttgttggttgagggtggctcaggctctggagttgccacacgaggtgcctcattagattcgctgtcagtggtgctactttcagtgtctgaatccgactcagagctgctctccgattcgctggagctgccagaacccccgctggcttgcactgcaggtgggggctggggagtggccaagggtgggttcacaggattattcctaggttttgccttttcaacagcctggtagagctcagtggcagtgcactgagtggtcaaggtcttcacaggctcaaggtcatcttcatcactgctcagcttcaggtcatcctcaagcatctttgtagaagctctggtggttgggtcattccacttttgtaaggtgaatcctggggtcagatgctgcgattcccgcaagatttcttcaacacagcttggatcactgggaaggcttacttcacttgtttggaggatggtgaactttggcagtttagtctttgaactggctgcactgggttttccatccaagagtgttccaaatgacagattcccaaagctgttctcaaattcaattgaaggtttcagtgttggtgagatgtccggtgcctggtcctggccatccatgggtctgacgtatgcagttggcttttgctgccccatgcttgttttgcagtaaagccctggtgggaagttttgaactgaaaggccactgctaggagctaataaagaggaagccactaggggagacccaggcgcttgcacggcgaattcagattcttccggtgaattggattgaaagatttctttgaaagcatcttctccactagaattagggttactgtcttcctttgcagatgggtttgactcttcaacttctccaatctggggctgttcagctgggtagacaaagaagtcttccagtttggcttgagactggtcctgtgtcaaagtctgcatcttgtttggctgaccactggcctggcttgccagtacagtgctagggttatgactatcacgtgaccactcaggttttgattttctgttgctgtgtattagagttgaattcagtatcacaacagaaggtggaggcattggtgctgaaggatgggtattatcctggtgaggtggaattattctgttcttttgttctggaaaaaagcttggttcatttttgttgttgggattctggggcacagaattctttggaattcccactaggtgattctgattagaatggttagttagcaaattcttcatttcatcatagtttccaagcgtgttctggactcggttggcaagtgcatcacctttgtttgtcttgtatggctccccaaaaagatcaaagcctgaagaaaagagatcgtcttcttgctggacttcttgattcctccgctcccattccctttttttaagtgcactacggtcttgttcatagtgacactgctgctccaagtcccagtctctgaaaaagtcgaatagatccatagcggccaggcggcggcggcgggcgggcgcctgtccctgatcgcagcgggtcggcgcggctctcggcacagctcgctggcggttctcggcggcccccggctctccagccctcccgcccagctaaaagtgtccgggccgcatcggcagcagcagcgggcgctggaggtgtctggtcctgtgctccggcgaggaagcggcggcagtggcactgggcgggcaagcgcctggtcgcccactcgggtccgctcggtccgcggtagcccgcgcacccagcgacccgacgctgcggcggcagccgctgcgggctcaggcgggctgggccgcccgcctggctggctgcgggccggcggcggcagcggcggcgggggcggccggggcagaggcagcggcgcggcgcggcagccggggcggcagcggcggcggcggcggcggcggcggcggcggcggcggcggcggcggcagcggctgcacaggcggcggc

SEQ ID NO: 18742 - RNA, 10372 nt, Homo sapiens
  source 1..10372: mol_type = other RNA
tgagtgtgtgtgtgtgagtgtgtgtgtgtgtgtatttaatgaaagcctcattatatactttagtttatgccttcttgttactgagcttagttttcttcgtactgggtggaaaaagaattattttggtttggattattgtttctgaatagtcatgcaattgatacagagatattctggtttgagttcagagctaaaacagtaagtagatacttttaactaaaaacaaatgttaacaaaaaacttagattccctaataactaaagtaaaattcttatgaacaacaatgtgaaggtgggagaattactgagtttccacgtcacataaaagaaaaacacagtaaattctggattgtgctattctccatagagttcccgtaaatactttatcctagttacatgtaaaagttacaaatagcatttgtaaatcaaaataatgatgacaataataataaaataaaaaacactcacttatctttttaaaaaatcaatcgtgagggttttctgagtgcccattttacctgtgagatatggaaggagatgatggaaccatctccattgatccatctctcctttcagctcaggagggcttcattcttctcagctattctcctgcttaaaacctaggcttccagggcaacccatacctctagggccttatcataagctttctacattcacacattgattcatatcttaaaactatgtaattgttttagtcatcgaagtgtgtgtgtaagggtgagtttgtgtgtgtgtgtctgtgtgtgtccacatgaacacatatattaaatatgaaccctctgactggctgcatccagtggcgtgttgaagcatttttgcccaggcttgcaagagccaactgcgtgcatctctttccaaccatgtgttcagtgacatcacagttggtagcttaaaatcatctaaagtggtagtatttatgccatggaaattggcaaatggtgcaaaccaggtgctttctattctcagcgagctggttgttaaacattttaccagcacaccactggttgcatgctaggctgaccaaatgagaagctagatcttgttctgggcaacacggcattaacttagcctcgttggagtgtctccaattttgcttactgtccagggtctccttcctcccaatttcataaacactgcagaaccacaacagggcttgagcatctggggtgcatttgactacccattgtcaccacattgggctctattctcagagacactttcgtagccacatgagtgatgcaggacaaaaccaaaaaggtaaagcatctgaaattccctccgaatatgacagctggcttcctgctgcagagactggagaacaatgagttccccaataggaacaaactattcccagctgaaagcatcagctggggcattcttcaggaggcttcccacagctggtctgcatgctgctgctcaccagcaactgctggcaggcaggcgagcttgagcttgctactgcagcatcctgtcaggggcctggacgtaggcttccttcacttcccccttccctcctcaaagtctgatacaaatcacagagccaacaaaattgaggtcactggcaaaagagtttgaaattttgaatgatttttattaaacaccattagtctacactgcacagttaatgaaacagcaaagctccaatctcttagaagaatgatgactgatcatggatctaaaaagcagttcagtgtcccctaacccaatgtgagcactatgaataattctttaacatctcatgtcagacgcaaaaaggggcaagaactgcaatctggctttgtggggcttccccaccccccacccccccgcccccacccccaccccctttctgccctccccacaatgcaattttcttttagctggtagattacagagtaaaatgtgatgattttggtaaagagggcttctatatttctgaggaggaggatggaaagagaattaatactttttccttcaccaaaaatatcagatggtaggattaatgtctgagaccggcctatctgattagtctcctgccagggtaaatgctgattatgaatacacagatgccacttctgttgttggagtctactaacactaaagagaaaatgaattagattttaattatgagaataaggccgtgcgagtgaaaatgagaaacaacaacaacaataacaacaacgatgaagaatttagtctgccagtcatgtaacagaacactgacaactggctcaataatttttccccacagaattaaatttgggggtgctgaattgacccattcatttgatactgtgtagctgtatcatcttgccacacatttttctcaatggggatagtgatgcttctctaagcaagcagttcattgctttactgagtagtcttacccagtgatccagtttggttctcccacctgccaactcatgcaggtgaattttatcatgtctgttgagaagtatgtgaggcttcaccctcacaactcaactgattctgccttcaaagatattttccaacctcaaactccaacttcaacctccgggatgcaaatttgcatgaaacagaatccaaattagatatctttgggaaagatatgctagaagagtatctttccaatgcagacaaaatctaatgaatttagtgatgtaatgtccaaatgaaaattcatccatttggaaactcaacaaaacacatttttagccaatggtttctaattttgcaacttgctttttgcctgaagattttggtcttttcatttccttacatggaaaaaaaggcatcccgaccttaagtcttttaaaagtagtagcagctaatctgcttttccaattatgtcatccaaatataaaactactagtattttcccaatgagattattaagtaattaacagtctacaggctggctaacaacatgcttacagctaaattctacccggaggaccacactagtaaacccttttcaaagtaatcctacctaccaaactcagacagttatatgacaaaaccactaaaaatccaaagttaattaaaaatacaaagccaagccaacatcataacacaaacttgtcaaactctctgtggttggagcttgggtgacaagtgaaggcgtagtggtggccctacctgggtcaagttgcagggctgagatcatttggtgtacttgctcagatggagcttccttttactctgccctctattctaacctccacgtgcttatttaagtgtgtctcaccaagcctccatcaagatctagaggcacgatctctcactgccatccacatgtctcatatccctcccacaaactggtatactgaagagattcatttgacagaatatctccatcccttagtccctcaaatagctgcacacctacgacacgcatcaccatttacactgtgatgaacagagtaactataaaacagcaacaatccttaatcatgaaactgaaagatgtcttatctcaagggataggaaggtaattcatcctccatgtttaattagttcctaagctgctttataaatgagtctactacataatcaagtggtgatccagagctcgattgtcagatttggtcactgtgctgcagacttggcacatattttacactcagtcaccagagatgacagagaatcctcttgcctccctgttgtatgtaagtagatataacaagtcactgaaactagaactacaagtctttcatccatgaggcaatatgcttgtttctctgggaaactgcctcaacattctaatgtctagtttctggatgtgggatttcaagaagaatctactcctaaatccatgatggtctaggattgtggtttaggttgaacttacaagtcaagccagtgggcttcattatatagtaatagccaggcactctacctggtaaaccatgataaagagacaacttgagtcactgcaaagtcatcagcttaatttttatatgtgacaccaaccttgggtgttcagagtctttaatgttatcatcattttcctcttttaagaggctcagaaaagattctttcaggtttcatttgtgagtgtttggatgcataagtgttgttgctgagactgtaaacataaagctcaaccacagtgggagcataaaaagtgctgggttcagctgcagggatgctcccatcagccatattaacaacatggcttcagccattggagtacaacttccacagccttatacaacaaaaggccttaaactcaaagatgaccagagcacagctcaagtctggctgttttgcaactggggatatatctaaccttgacaatgagagtgcagagtcatcacctgctgtttctatcatggacctgcatggctggctttaataatcacacaagtttgcatctttcatgtgcatatctattatttatctggtcataactcagtgaacagaatttgataacccagcatattaaaggctacatggaattatataccagcaggtaattaccagtaagtaatgcatggatagtgtttaccccaagtgtaagaatcttctggtgagctggaacatcaaaaatgatatttacattgtgatgtttagggacataaaatgaatgtgaaggatcataagggggtagtcacaaccagtgagaaatgtctccaaattaggtgaatggttcccaatgtttagggctctttcaaagcatctcaaggtgaagcactaccccacgactcattttaaaaaaataaaagttagctactatttagagagtttggagttttcttagaaattttcatggaaatgattcacaataatatggactttaataaaaggagtaattgtaattcagtcaaaagttaatgagccaaacaaaggaaagggaaacacagataagagaaaaaagaaagtagaaaacagaaaacctataagagagaaaatgtgaataataattgaggaagtccagattttcaagccactaggaagaaaactgtatatcattacttctaggtagtgataccttgacttttgttcccatagatttgagcaaaatacaatttaaaaatcctgccagttatggacccacttaccaactgtgtaaatgttgttgttgcaaaggaggcagaggtgtgaattccttgttggacactttccagacctctcttaactcccacttgtaagtctagagtgtagcattttggctactaaggcatgcatcaaccaaactgttcttcaaaaggacagctttgcacacagagaaccccaggtgaggatttacacttcaaataatggagttgaaaaacactgatgccagctgatgcctaaaacttgtcaaaataaatgtcaccctttcttcttatcattaaaattaacaaaatagggaatcaggaaagggatgctaacaagaaagtcctctggttgtgtggcatagcatctttttaagagtagcattgctatgctcatttattttcttgatactcttgattttatgatgttgctacaacatctaaccagtgggttttgacaatgaaaattctcacctgaagattgaatctgtgggatacacaaaagtttgacagattctgaaatatgttcttttctgggtataagagtagagtttgggggatggtcccttgtgtctaagttctcatgtatatgtaagaccacttgttgcatttctcaggagcctgtctttatcacaagtgcttcccattctttgttttgggtagtgtgggcttaaaacaatattgtagggactgtcattccataaagcacaaaaagatggtggaatctgagaaatgcatatcaaatgctaaaagaaaaaaaatgactaagtaataaaacgtacactgcccttaagttgtagtgtcaacttacaatgacttctgttttttacagataacaaaagaagcataaaaacaaacataaccaaagagaacgttccccagtgagtggagttccaccagtgaccatcagtgcgctggtagaggtagagtgatgggtcgtgatgctagagatctgagaacacccactacaacaagtgggcatcgatgcgcagccaacacagtccttggcgaacgtagcggacaagattggtcatgctgctgtgctgggtcagaggccccatcagcgtgtccagatcaccaaagaattctttgttttctcttgtcagtttgtcggccatatcccagtgttcatagccccgtaacacattgctagtgatgttgacgtggctggcagccatgtggtgaatgcgctggggaatggtgactgggccattgttacagttccccattgcgttgatgggggagacgttgttgagagacactggggatggagtgttctttccattgcttacccatggagagggtatctgtgcgacttttgaagcattttgcttaaaatattccatcagtgatctggagtacttcatagcatggtccttcttcagcttaaacattctcaaatagaggagtgataaacatcggtagcatagtactgctagctttttgtccccatccgaagccaagggacttgcaaagttcttcagcctcattgcatacctgaggagctccacagtctcagagtacatggtgtatggggactttgcttccagagggtcgcgttccatggcattgccacattcagtgaaggagagggcggcatcagcataattcacagctttgccaaatttctcgaacagtgcatcagctttgtgcttcagcttcttagcttcttgcatgtaataatcagcattgtgaaccgagtcatcaaaagtgagcttgggtctccggacattagtgctgctgctggatagaaggggcagagccgcccaggacgtcatctccaggtgactgctatccatgaggccagtagtgatggtagaggtgatggtggaaatggtagtggtagtagttgtggtggtggccgtggcggtggcagtagctgtgacagtggtggtgacaatggcagtagcagtgacagtagcagtggcaatagcagtattggtgacagtgatggtggcagaggatgccttttttggagtgtctccctcatttaccgatatccctttgaaagtagcacagaatttgccttcagttctcttaggtttggtagatgtgatttgtccagtcatggcgatgtttttgtcttgaccaaagggaccattattgccactgacatttctgcggcgtggagggtcctctggcagtggggaaagtggaggaggaaatagtttttcttcctttcttctatttgctctcctggatgaattattttctctagtgttgggaggcttgtggggtggggctggtgagatgcaaggagggagcaagcagatagttgtggcctcctccaggcgctgcttcttctcagggatcttctctgcaacttctattggcttgtgcttacgtttgcccttaggggctggtttctccacagctgtgacagctgtctgacgcttgggttttgtggcagtctccttgtggtctggcttggcaggtgctgcatggagtgagctgtggccaggtactctagagagtaagtcaaggtcaatcttcacccagaggtttttcaggttctcatgatctcgcagaggggacaggatttcagtttgcatgacaggaataggtgaaaatgttggctcttcattactgatggataagttgttgttgctgccactgctactcattaaggtgctgagggtcaggctggcaccacagatttccttggatttggcagtattacctccagaaataatgcacggaggcaggactttgatttgcagggtctcttcctgatctgtgttggagtcagatgtagatgaatctgtttcaatgaattcccgagactttggcacaatcttgccaggccctctgtacttcttcttctcgggagccaaagggatgttaggtcttggttctttcctaggggctggtttgtgggcagtggctttgttgcggcctcttggtgggtcatgaagctccacactttctttttctttgggagtgctgctggtaatatttggtttgggccaggtaaactcgtcagtgctggtgttcttctcaacttttttgggctgttttttcccaattgtcctttgagacactgtctcactagttgttgacaacttatgcttcaaagcctttgtttctggaattttctgagtgggccgtggacgggctttctccctaatgagactgaggagaggcctttctttgggttcagctgggacctgactggcattcgtcttcactttcatctggacttccattggttggatgattggaggaggcagagaaatagtctccatgggtgtttcattttggccacaaataaaagacttgttctgggatgtcactttgttaagccatttatccagttgccacttgttggttgagggtggctcaggctctggagttgccacacgaggtgcctcattagattcgctgtcagtggtgctactttcagtgtctgaatccgactcagagctgctctccgattcgctggagctgccagaacccccgctggcttgcactgcaggtgggggctggggagtggccaagggtgggttcacaggattattcctaggttttgccttttcaacagcctggtagagctcagtggcagtgcactgagtggtcaaggtcttcacaggctcaaggtcatcttcatcactgctcagcttcaggtcatcctcaagcatctttgtagaagctctggtggttgggtcattccacttttgtaaggtgaatcctggggtcagatgctgcgattcctgtcctgggatggaaaaggtgctctgctcagagtgtccagcagtatgcatggaagtgagaggagtaggccaggaatgggtcatctcccgcaagatttcttcaacacagcttggatcactgggaaggcttacttcacttgtttggaggatggtgaactttggcagtttagtctttgaactggctgcactgggttttccatccaagagtgttccaaatgacagattcccaaagctgttctcaaattcaattgaaggtttcagtgttggtgagatgtccggtgcctggtcctggccatccatgggtctgacgtatgcagttggcttttgctgccccatgcttgttttgcagtaaagccctggtgggaagttttgaactgaaaggccactgctaggagctaataaagaggaagccactaggggagacccaggcgcttgcacggcgaattcagattcttccggtgaattggattgaaagatttctttgaaagcatcttctccactagaattagggttactgtcttcctttgcagatgggtttgactcttcaacttctccaatctggggctgttcagctgggtagacaaagaagtcttccagtttggcttgagactggtcctgtgtcaaagtctgcatcttgtttggctgaccactggcctggcttgccagtacagtgctagggttatgactatcacgtgaccactcaggttttgattttctgttgctgtgtattagagttgaattcagtatcacaacagaaggtggaggcattggtgctgaaggatgggtattatcctggtgaggtggaattattctgttcttttgttctggaaaaaagcttggttcatttttgttgttgggattctggggcacagaattctttggaattcccactaggtgattctgattagaatggttagttagcaaattcttcatttcatcatagtttccaagcgtgttctggactcggttggcaagtgcatcacctttgtttgtcttgtatggctccccaaaaagatcaaagcctgaagaaaagagatcgtcttcttgctggacttcttgattcctccgctcccattccctttttttaagtgcactacggtcttgttcatagtgacactgctgctccaagtcccagtctctgaaaaagtcgaatagatccatagcggccaggcggcggcggcgggcgggcgcctgtccctgatcgcagcgggtcggcgcggctctcggcacagctcgctggcggttctcggcggcccccggctctccagccctcccgcccagctaaaagtgtccgggccgcatcggcagcagcagcgggcgctggaggtgtctggtcctgtgctccggcgaggaagcggcggcagtggcactgggcgggcaagcgcctggtcgcccactcgggtccgctcggtccgcggtagcccgcgcacccagcgacccgacgctgcggcggcagccgctgcgggctcaggcgggctgggccgcccgcctggctggctgcgggccggcggcggcagcggcggcgggggcggccggggcagaggcagcggcgcggcgcggcagccggggcggcagcggcggcggcggcggcggcggcggcggcggcggcggcggcggcggcagcggctgcacaggcggcggc

SEQ ID NO: 18743 - RNA, 10297 nt, Homo sapiens
  source 1..10297: mol_type = other RNA
tgagtgtgtgtgtgtgagtgtgtgtgtgtgtgtatttaatgaaagcctcattatatactttagtttatgccttcttgttactgagcttagttttcttcgtactgggtggaaaaagaattattttggtttggattattgtttctgaatagtcatgcaattgatacagagatattctggtttgagttcagagctaaaacagtaagtagatacttttaactaaaaacaaatgttaacaaaaaacttagattccctaataactaaagtaaaattcttatgaacaacaatgtgaaggtgggagaattactgagtttccacgtcacataaaagaaaaacacagtaaattctggattgtgctattctccatagagttcccgtaaatactttatcctagttacatgtaaaagttacaaatagcatttgtaaatcaaaataatgatgacaataataataaaataaaaaacactcacttatctttttaaaaaatcaatcgtgagggttttctgagtgcccattttacctgtgagatatggaaggagatgatggaaccatctccattgatccatctctcctttcagctcaggagggcttcattcttctcagctattctcctgcttaaaacctaggcttccagggcaacccatacctctagggccttatcataagctttctacattcacacattgattcatatcttaaaactatgtaattgttttagtcatcgaagtgtgtgtgtaagggtgagtttgtgtgtgtgtgtctgtgtgtgtccacatgaacacatatattaaatatgaaccctctgactggctgcatccagtggcgtgttgaagcatttttgcccaggcttgcaagagccaactgcgtgcatctctttccaaccatgtgttcagtgacatcacagttggtagcttaaaatcatctaaagtggtagtatttatgccatggaaattggcaaatggtgcaaaccaggtgctttctattctcagcgagctggttgttaaacattttaccagcacaccactggttgcatgctaggctgaccaaatgagaagctagatcttgttctgggcaacacggcattaacttagcctcgttggagtgtctccaattttgcttactgtccagggtctccttcctcccaatttcataaacactgcagaaccacaacagggcttgagcatctggggtgcatttgactacccattgtcaccacattgggctctattctcagagacactttcgtagccacatgagtgatgcaggacaaaaccaaaaaggtaaagcatctgaaattccctccgaatatgacagctggcttcctgctgcagagactggagaacaatgagttccccaataggaacaaactattcccagctgaaagcatcagctggggcattcttcaggaggcttcccacagctggtctgcatgctgctgctcaccagcaactgctggcaggcaggcgagcttgagcttgctactgcagcatcctgtcaggggcctggacgtaggcttccttcacttcccccttccctcctcaaagtctgatacaaatcacagagccaacaaaattgaggtcactggcaaaagagtttgaaattttgaatgatttttattaaacaccattagtctacactgcacagttaatgaaacagcaaagctccaatctcttagaagaatgatgactgatcatggatctaaaaagcagttcagtgtcccctaacccaatgtgagcactatgaataattctttaacatctcatgtcagacgcaaaaaggggcaagaactgcaatctggctttgtggggcttccccaccccccacccccccgcccccacccccaccccctttctgccctccccacaatgcaattttcttttagctggtagattacagagtaaaatgtgatgattttggtaaagagggcttctatatttctgaggaggaggatggaaagagaattaatactttttccttcaccaaaaatatcagatggtaggattaatgtctgagaccggcctatctgattagtctcctgccagggtaaatgctgattatgaatacacagatgccacttctgttgttggagtctactaacactaaagagaaaatgaattagattttaattatgagaataaggccgtgcgagtgaaaatgagaaacaacaacaacaataacaacaacgatgaagaatttagtctgccagtcatgtaacagaacactgacaactggctcaataatttttccccacagaattaaatttgggggtgctgaattgacccattcatttgatactgtgtagctgtatcatcttgccacacatttttctcaatggggatagtgatgcttctctaagcaagcagttcattgctttactgagtagtcttacccagtgatccagtttggttctcccacctgccaactcatgcaggtgaattttatcatgtctgttgagaagtatgtgaggcttcaccctcacaactcaactgattctgccttcaaagatattttccaacctcaaactccaacttcaacctccgggatgcaaatttgcatgaaacagaatccaaattagatatctttgggaaagatatgctagaagagtatctttccaatgcagacaaaatctaatgaatttagtgatgtaatgtccaaatgaaaattcatccatttggaaactcaacaaaacacatttttagccaatggtttctaattttgcaacttgctttttgcctgaagattttggtcttttcatttccttacatggaaaaaaaggcatcccgaccttaagtcttttaaaagtagtagcagctaatctgcttttccaattatgtcatccaaatataaaactactagtattttcccaatgagattattaagtaattaacagtctacaggctggctaacaacatgcttacagctaaattctacccggaggaccacactagtaaacccttttcaaagtaatcctacctaccaaactcagacagttatatgacaaaaccactaaaaatccaaagttaattaaaaatacaaagccaagccaacatcataacacaaacttgtcaaactctctgtggttggagcttgggtgacaagtgaaggcgtagtggtggccctacctgggtcaagttgcagggctgagatcatttggtgtacttgctcagatggagcttccttttactctgccctctattctaacctccacgtgcttatttaagtgtgtctcaccaagcctccatcaagatctagaggcacgatctctcactgccatccacatgtctcatatccctcccacaaactggtatactgaagagattcatttgacagaatatctccatcccttagtccctcaaatagctgcacacctacgacacgcatcaccatttacactgtgatgaacagagtaactataaaacagcaacaatccttaatcatgaaactgaaagatgtcttatctcaagggataggaaggtaattcatcctccatgtttaattagttcctaagctgctttataaatgagtctactacataatcaagtggtgatccagagctcgattgtcagatttggtcactgtgctgcagacttggcacatattttacactcagtcaccagagatgacagagaatcctcttgcctccctgttgtatgtaagtagatataacaagtcactgaaactagaactacaagtctttcatccatgaggcaatatgcttgtttctctgggaaactgcctcaacattctaatgtctagtttctggatgtgggatttcaagaagaatctactcctaaatccatgatggtctaggattgtggtttaggttgaacttacaagtcaagccagtgggcttcattatatagtaatagccaggcactctacctggtaaaccatgataaagagacaacttgagtcactgcaaagtcatcagcttaatttttatatgtgacaccaaccttgggtgttcagagtctttaatgttatcatcattttcctcttttaagaggctcagaaaagattctttcaggtttcatttgtgagtgtttggatgcataagtgttgttgctgagactgtaaacataaagctcaaccacagtgggagcataaaaagtgctgggttcagctgcagggatgctcccatcagccatattaacaacatggcttcagccattggagtacaacttccacagccttatacaacaaaaggccttaaactcaaagatgaccagagcacagctcaagtctggctgttttgcaactggggatatatctaaccttgacaatgagagtgcagagtcatcacctgctgtttctatcatggacctgcatggctggctttaataatcacacaagtttgcatctttcatgtgcatatctattatttatctggtcataactcagtgaacagaatttgataacccagcatattaaaggctacatggaattatataccagcaggtaattaccagtaagtaatgcatggatagtgtttaccccaagtgtaagaatcttctggtgagctggaacatcaaaaatgatatttacattgtgatgtttagggacataaaatgaatgtgaaggatcataagggggtagtcacaaccagtgagaaatgtctccaaattaggtgaatggttcccaatgtttagggctctttcaaagcatctcaaggtgaagcactaccccacgactcattttaaaaaaataaaagttagctactatttagagagtttggagttttcttagaaattttcatggaaatgattcacaataatatggactttaataaaaggagtaattgtaattcagtcaaaagttaatgagccaaacaaaggaaagggaaacacagataagagaaaaaagaaagtagaaaacagaaaacctataagagagaaaatgtgaataataattgaggaagtccagattttcaagccactaggaagaaaactgtatatcattacttctaggtagtgataccttgacttttgttcccatagatttgagcaaaatacaatttaaaaatcctgccagttatggacccacttaccaactgtgtaaatgttgttgttgcaaaggaggcagaggtgtgaattccttgttggacactttccagacctctcttaactcccacttgtaagtctagagtgtagcattttggctactaaggcatgcatcaaccaaactgttcttcaaaaggacagctttgcacacagagaaccccaggtgaggatttacacttcaaataatggagttgaaaaacactgatgccagctgatgcctaaaacttgtcaaaataaatgtcaccctttcttcttatcattaaaattaacaaaatagggaatcaggaaagggatgctaacaagaaagtcctctggttgtgtggcatagcatctttttaagagtagcattgctatgctcatttattttcttgatactcttgattttatgatgttgctacaacatctaaccagtgggttttgacaatgaaaattctcacctgaagattgaatctgtgggatacacaaaagtttgacagattctgaaatatgttcttttctgggtataagagtagagtttgggggatggtcccttgtgtctaagttctcatgtatatgtaagaccacttgttgcatttctcaggagcctgtctttatcacaagtgcttcccattctttgttttgggtagtgtgggcttaaaacaatattgtagggactgtcattccataaagcacaaaaagatggtggaatctgagaaatgcatatcaaatgctaaaagaaaaaaaatgactaagtaataaaacgtacactgcccttaagttgtagtgtcaacttacaatgacttctgttttttacagataacaaaagaagcataaaaacaaacataaccaaagagaacgttccccagtgagtggagttccaccagtgaccatcagtgcgctggtagaggtagagtgatgggtcgtgatgctagagatctgagaacacccactacaacaagtgggcatcgatgcgcagccaacacagtccttggcgaacgtagcggacaagattggtcatgctgctgtgctgggtcagaggccccatcagcgtgtccagatcaccaaagaattctttgttttctcttgtcagtttgtcggccatatcccagtgttcatagccccgtaacacattgctagtgatgttgacgtggctggcagccatgtggtgaatgcgctggggaatggtgactgggccattgttacagttccccattgcgttgatgggggagacgttgttgagagacactggggatggagtgttctttccattgcttacccatggagagggtatctgtgcgacttttgaagcattttgcttaaaatattccatcagtgatctggagtacttcatagcatggtccttcttcagcttaaacattctcaaatagaggagtgataaacatcggtagcatagtactgctagctttttgtccccatccgaagccaagggacttgcaaagttcttcagcctcattgcatacctgaggagctccacagtctcagagtacatggtgtatggggactttgcttccagagggtcgcgttccatggcattgccacattcagtgaaggagagggcggcatcagcataattcacagctttgccaaatttctcgaacagtgcatcagctttgtgcttcagcttcttagcttcttgcatgtaataatcagcattgtgaaccgagtcatcaaaagtgagcttgggtctccggacattagtgctgctgctggatagaaggggcagagccgcccaggacgtcatctccaggtgactgctatccatgaggccagtagtgatggtagaggtgatggtggaaatggtagtggtagtagttgtggtggtggccgtggcggtggcagtagctgtgacagtggtggtgacaatggcagtagcagtgacagtagcagtggcaatagcagtattggtgacagtgatggtggcagaggatgccttttttggagtgtctccctccgatatccctttgaaagtagcacagaatttgccttcagttctcttaggtttggtagatgtgatttgtccagtcatggcgatgtttttgtcttgaccaaagggaccattattgccactgacatttctgcggcgtggagggtcctctggcagtggggaaagtggaggaggaaatagtttttcttcctttcttctatttgctctcctggatgaattattttctctagtgttgggaggcttgtggggtggggctggtgagatgcaaggagggagcaagcagatagttgtggcctcctccaggcgctgcttcttctcagggatcttctctgcaacttctattggcttgtgcttacgtttgcccttaggggctggtttctccacagctgtgacagctgtctgacgcttgggttttgtggcagtctccttgtggtctggcttggcaggtgctgcatggagtgagctgtggccaggtactctagagagtaagtcaaggtcaatcttcacccagaggtttttcaggttctcatgatctcgcagaggggacaggatttcagtttgcatgacaggaataggtgaaaatgttggctcttcattactgatggataagttgttgttgctgccactgctactcattaaggtgctgagggtcaggctggcaccacagatttccttggatttggcagtattacctccagaaataatgcacggaggcaggactttgatttgcagggtctcttcctgatctgtgttggagtcagatgtagatgaatctgtttcaatgaattcccgagactttggcacaatcttgccaggccctctgtacttcttcttctcgggagccaaagggatgttaggtcttggttctttcctaggggctggtttgtgggcagtggctttgttgcggcctcttggtgggtcatgaagctccacactttctttttctttgggagtgctgctggtaatatttggtttgggccaggtaaactcgtcagtgctggtgttcttctcaacttttttgggctgttttttcccaattgtcctttgagacactgtctcactagttgttgacaacttatgcttcaaagcctttgtttctggaattttctgagtgggccgtggacgggctttctccctaatgagactgaggagaggcctttctttgggttcagctgggacctgactggcattcgtcttcactttcatctggacttccattggttggatgattggaggaggcagagaaatagtctccatgggtgtttcattttggccacaaataaaagacttgttctgggatgtcactttgttaagccatttatccagttgccacttgttggttgagggtggctcaggctctggagttgccacacgaggtgcctcattagattcgctgtcagtggtgctactttcagtgtctgaatccgactcagagctgctctccgattcgctggagctgccagaacccccgctggcttgcactgcaggtgggggctggggagtggccaagggtgggttcacaggattattcctaggttttgccttttcaacagcctggtagagctcagtggcagtgcactgagtggtcaaggtcttcacaggctcaaggtcatcttcatcactgctcagcttcaggtcatcctcaagcatcgatttgaaagacactgactttgtagaagctctggtggttgggtcattccacttttgtaaggtgaatcctggggtcagatgctgcgattcccgcaagatttcttcaacacagcttggatcactgggaaggcttacttcacttgtttggaggatggtgaactttggcagtttagtctttgaactggctgcactgggttttccatccaagagtgttccaaatgacagattcccaaagctgttctcaaattcaattgaaggtttcagtgttggtgagatgtccggtgcctggtcctggccatccatgggtctgacgtatgcagttggcttttgctgccccatgcttgttttgcagtaaagccctggtgggaagttttgaactgaaaggccactgctaggagctaataaagaggaagccactaggggagacccaggcgcttgcacggcgaattcagattcttccggtgaattggattgaaagatttctttgaaagcatcttctccactagaattagggttactgtcttcctttgcagatgggtttgactcttcaacttctccaatctggggctgttcagctgggtagacaaagaagtcttccagtttggcttgagactggtcctgtgtcaaagtctgcatcttgtttggctgaccactggcctggcttgccagtacagtgctagggttatgactatcacgtgaccactcaggttttgattttctgttgctgtgtattagagttgaattcagtatcacaacagaaggtggaggcattggtgctgaaggatgggtattatcctggtgaggtggaattattctgttcttttgttctggaaaaaagcttggttcatttttgttgttgggattctggggcacagaattctttggaattcccactaggtgattctgattagaatggttagttagcaaattcttcatttcatcatagtttccaagcgtgttctggactcggttggcaagtgcatcacctttgtttgtcttgtatggctccccaaaaagatcaaagcctgaagaaaagagatcgtcttcttgctggacttcttgattcctccgctcccattccctttttttaagtgcactacggtcttgttcatagtgacactgctgctccaagtcccagtctctgaaaaagtcgaatagatccatagcggccaggcggcggcggcgggcgggcgcctgtccctgatcgcagcgggtcggcgcggctctcggcacagctcgctggcggttctcggcggcccccggctctccagccctcccgcccagctaaaagtgtccgggccgcatcggcagcagcagcgggcgctggaggtgtctggtcctgtgctccggcgaggaagcggcggcagtggcactgggcgggcaagcgcctggtcgcccactcgggtccgctcggtccgcggtagcccgcgcacccagcgacccgacgctgcggcggcagccgctgcgggctcaggcgggctgggccgcccgcctggctggctgcgggccggcggcggcagcggcggcgggggcggccggggcagaggcagcggcgcggcgcggcagccggggcggcagcggcggcggcggcggcggcggcggcggcggcggcggcggcggcggcagcggctgcacaggcggcggc

SEQ ID NO: 18744 - RNA, 23245 nt, Homo sapiens
  source 1..23245: mol_type = other RNA
tgagtgtgtgtgtgtgagtgtgtgtgtgtgtgtgtgtgtgtgtgtgtgtgtgtgtgtgtaattcaaggtaaagttttcattattaaagactgcccaataatctctctcaggacactgaagcagaagctagaagatgccatcagagacccagtagccagatgtagctgctgattacgaaagacaggatctacactggctactgagccattgagggtacctacaccttccagcagctgggtgatcctttgccttctggggaggggctctgtggaagaaaaaagaagatatcagatttcaattgcacattttctttggatcatgaattgacattttgacaatattcccatgtacgtaattttaaacaacctctggatttatttacttatccaacagatactgactgagtgacattaaataaagtgccacatattttcttaggtgctggagatccagcagcaaacaaaaaaagtggaaaatctctatacttctacagcatacatgattccttgtgacaaaatctacaatcaattatttggtatgttttgcagtaaaatggaaatatacacaagagaaaaacaaacaagcaaacaaaaaaccaatctaccattttattgtggcttggagcatttttgttgcttcctgtcactttaacttgggtaatctagcaatgatgcacatatgtaaagtaaattgcagttaaaaaattctttcgtgttacgaactgaggataatacagttattttaccaaatatctcaaacaccaaagaaaattacagaaaatgcatattataataaatattcaaagcaggtgctcactagcatgtcagttccaagctttcctcccatgatacaatgaaggtaacaaaataagtcacaggattggtgttctctttgctattcatttatccaccccagaaatacttactgagtaccttcaataagtacctttcagtaccttactgaaatacttctgcgtgctttattccaggcactgggaatgcaacactgaacaaaatccttgcactcacggaagtttaagtctaagatttaaggaaagggtagaaaaagactgaaaaaaacctccatagatatggacggtcatttcatagagtaatgaaacagttaagaggaatgctattttcgataaggtggctaggaaaagcctcactgagggcctggcatttgagtggattcctgaagtaggaggagaagaatcatgtacatacctggggtgggaaaggacaccacagggagaggcaagagtcagaacaaaaagcactgaaacaggaaaaagcctggtatcttggacaaggtgttcttttattagcacatgaccacatggccaattattgtttcctacttttaggattattctagaaggtaaatgactatgcaacttttctccaagtacacgtcttagaatcctttgctgtgaatttaaaatgcttcagctatcacttagaaaagatttaataaagctactgtcaattggaaactagtaccatttgatcggacatgcagctataccacagtatgacacacacatatttatcaccaagagaaaagtggctttttaaaaatgtgttagctataagaaaagataaccagctttctgggagctctaaatatatacatatctagggaatgatttaactatttaatcacagatgtctaattttaagaggcaactcacttgccaaattatagtaatagtgcttcaccagtgtggttagctcttggtgggggaggataagggtggaatttacaaggtgaagcaggggtttttttgattgcttgcttttttttctctttaaataagttaaggccaatcccatctatgaagtatattttggcactgcctacaaaccagagcatacatactgaagtgggggaaaagaccgtttatataggtttggctaagtcttaccctcaatgtaaaataaagcatttgtagaacacacaaacttacatttcataaaccactaaaactaactgttcataactctacttttatgaataagactaacaattaaagtgaggcaagggtttagtgtggtcactttcaatgccaaaatacaaaagattatcttttataaatctttacatttagatgagaaaaggtaaatttttaattctcaaaggtatctattctccacatcttagtactaaagttaaggtggtcttttgccccttgttttaaatttaatctaggtaatacaaataggaaaatctgtaaataaaattttattaaaggttattctgtaaattagtgtcaaccactaaacaatactatacagttttaagtttattaaaaacacaaagaatagaatatgtagaatatataacaccatagaatattaaccaataatgcattttcagtttaaaaataaaaggaaaagaaaagaaataggttcaaactagaaatgttgagttatataattctgttatctaacaattaagatgacaactaagccccaagggtgagtgataggactgtaaccaaggtacttctgctcaagtcctagtcacactgcaaacaaacaaaacaaaaataataataaacaaaaactcccatacattctggctaaagaccatttatttgaggtatgagaaagagtttaaagggagggaaagactattaaaagttaagcctgccacctgctgttggaaggcctgctttgaactgggataaagaccatttcttgaaatgttaacctagaatttgaagagcttacactccacacggttagaacaggggcaacctatacaccaaaccaagaagtaaagaaacccattgatgtttaaagctacactgagagagataaaagtcacattcgcatcaaagttctactggaaatgaaagaaatgctgcttcgtgcgtcattctactgaaggaagagtagaattactctgtcttttaaactgattacctggacaattctattttgcccccaaaaagcatctctgactttagaaattatcatttttagaaagaaattttgaccctagggactatatgtggaagtaaatgaagagagatgaacgatttcacagcattgccagaatgctaactttaccaagtcaaaattgtctaattcactgtttttaacacaaatgtgaaagaatctatgcttctttgagtaaaagaacttccagatgctttccagttccatgattttctataacctcacaaagtctggccccacatgtccccctaaaccccatccatgatatttcacatatttttgttcatgcaccagtagttttctgtaactaaataggaatagagtcaaattctatcacaatcatgtttagggatttgacagagcataagccagtccactattctaatgaagtcagagtttactttagaagtgaacaaaaactgccacccacagtgtatatctcatgttaagtgattcttaacatatacacaaacacagacacaaaaccaaagggatacaatgaaactttgagagatgttgaatacatccattaccttgattatggtgatggtatcacaggtgtttgcatatatccaaactcatgaaattttccacatgaaatatgtgcagttctttatcaattatacttcaataaagctgtttttttttttaaaaaaagctgcctcccacaccgttaagaacaaaaagtccaattaactctaactgtaggccagggaagaaatgcacccatgtatacacagtgcgccacagggtgaaattatgctagaggagaaatcagccttttaaatacaggtgtctaattaaagtatgttcttatgaacttggattccttctgtgttatgttatgttagagcaactgagccagggtatcaccataaccgggcacgtggttgaaacccgtccagctcttgcatacctgagatcctgtgactacactgaccaaaaacatttataccagctgatggtcacttgattctcacatctctctatttagtaaattgctccgcaagccaacttgaagactgaggtgaacattctctgggacgttcctgctgaagacatttttttaaaagacattgcccctgccagataattctagtctgaacaggcctcagaagggactggttggcacaagatcctaaaacaagcttctaaaggtgaaaccactcagagcccataaagacagactcagactagttttttaaaaactaatatttaacaattaggtgcatgcctttaatccttctcaacgaaaaacaacattttttaaacaatcaatagatgaaaacatgaagcattttactcattgcaaacactcagaggaaaaggatagttttaacctaagtaacaaacagtctttttatggacaagtttcagaaattaattgccctaaatccatgtacatatatatctctctttgtccctctccccacactctggaagaaaaccctaaggcattctctacatacaatgtcagcagtgtgcaacgatggtgaggaattcttgtcgtttttaaataaaagaaagaggaaaataatttgcattccatcaatgataagtaaaaacaaaagaaggacgtcaaaataaagtaacttctctgagcttgtgaatagcagaaaaaccagtcagttctctcaagaattcatgacttagagacttatttagtgacaattaacccattactactctatactattaccgaggcctttctgtggatttggtctcatttttaagccttgtgctattttctaaaggcatcaacatcgcacatgtctaccattgcaaccttcatttataatcagatctctaccaagcctctgcttttggcactgtacagaacttcttttgtcatacaatgttcttatggtacaaaattctttgtgtcgtcttccttgaatcttcccatcaagtttccctctcctcagatggactgatggaggagcaaaattcggcttctgaacactgcctgacaagcacttccctccctgcaaggcccagctctcttataggatgctaagggaccttcctggattcctctggaaagttagctgcatactactgggggctggttcccagatcactgagtctgtggtctcagccagaaacacaagacacattgctcttcaatttgtttagaaatgtgtctccctgtgagaatatgtgctctttgagggtaagaatcagtcccataattttgagattccccaggtaccagcatagtacactagatcatagtcaccttttagtaaatatttgtcaaataaagaaatgtgagtgaatagacagtaaaatgcctgacacctatactgatacatttcaaaaaacaacaaacacaaacacacacacacacacagtggaagactatctccattcagggaaactcttgtatttcttcatcctttaaacatttcttgctttctctcttagttttatggtagctttctgtaagatttgtgggtgcttataagatcatgctatttgtaaaagagtgtatgttccttttaacagaagtatggactagtgaaagcactgtcttagagtgtgtttgtgtaccatcacaggtttgtagcacagaagggtcctcagggaaataaaatctactccagtaaaatgataaaactaagacaaatgaacaggtaatgagggaagaccagaaagagaacatccatatatacagtttcttttgcttatgatggttatcagaagctcaaccacattaggtatcaattattatgagttctatgacagtatgtggacttttaaaattaagtggcttatataaatagctcacaccacaatggaagagaaaggaagatagttagcagaagaagtgtgaagattcggaaagactaataaaaatgatttttaaatgatgaagggctaaatgtatttcccgcagatgctatttgatgacctatcaggtacaaaacacacacacacacacacacacacacacacacacacacacttcagcaaagaggaacaggatgaaaacatggattctacttgtgtaacaaagagaaaatggaaacgctaattaagatttttaaagaaagaatgttctaaaatgtgttaaacgaagggaaagaggggaaatagatattttcaaactacgaagaaagactacagtataaagacctaacctacaagtccagtatttgctcccagagtggctgccacacagtggacgtgtgatcagttcttcaacaggttgtaaggaaacctcaactgttttggaggaaataactcggtacaccccaaggaccatgcaaagccttgataatagcacaacagcatccttctaccccttcttctctccttattggttgatgctggactgtatttgtgctgacagtggaaggttttttgacaacgtatggacagttctatagagcaaaatataagtatctagaaaaacaacatcaatataattaaaaatcagattaaaaattaggattcaaaacactaacaaagaggaaaatggcaaaatatcaagcactcagcttacaattggagatggtctacaacatgacagtctggaatgtaaaaaggaagcaggatattgaagagggagcaccaccgcaagtgagaaaagagccagggagagagacgtcagtcaatacaccagaagagaaaatggacatagggaagcccaatgcccagatactcatcaatgaggcaagagcttcatgggcgcccactattattaactaggtagaataagaagtttaccaggtagggaaaaccagaaggtggggaagggaaggaggctgaggagtaactcttggaggtttaaaaaaaatgttagaaaaggtgagcatccggagtccatgacaaagcgaagattattcataggcctgggcaaagtcaagagatgaaggaaggaagtctttcttcctgtgcggggtggggagagcagcagcagcaaactttatcactaggttgaaaggggaaataacagaaacaaaactgctgtttgtattgatggcagtcacacaggggaaatctggttcctctttctatgagtgaagaaagaggtcaggggaggtacttggcactaaaggatgatataaccttgaaaggactggctcagggaggacaagagaatggtgtgtgtgtgtgtgtgtgtgtgtgtgtgtgtgtgtgtgtgtgtgaaggggagacctggtggagtgtgaatggcaatatgctatgggagtcgttttcactcaaaaaggaatagcaaaaccctctcatacagagaaaatgacagggcgcaaggagctcaaaaatgaagaggagccttccacttctaacaagaacacactagatgtaaattggcaatgctgaaagagcagtgagtcccagagccagaaggaactttcctaaggtatccagcccgtggatagtctaaatgtcccacgtagatgtgacaagccaggaatgatcccaatttacctagctccagaattgcctgatcttcttcttgactcaatgcccccaacctcacattcatccccttgcttcccatttctagctagtaggtaacagcactgagcccgttcaaatttctcacagacagtctctattcattctgacattatctctccagtaagtcctactctggttatcaaactttctgtagtctggagaacaaacaaatccctaatatggtcattcttttcatgctgagagatcaaactcatcctattactgggatcagtaatagtaaatgcaaccctgacaccgacaggagagagtcgtcaggtacattaccacttttcttcacagctgcccctatgaatgccatgaaggaccacggaattagggatggaataaattcgaggatttgatgaaaaacaaaacaaaaaaatagggctccctttgattgtcatccttagacaaaatttgatactctttgcactaccatatgattatatcccctgattttctaagattaaagtccattagagttagaaattggaactctcaagccgaagtcaagaaaacaaatcatgtctggttttagaggtgccagaatgatacaatggactttggagacttcggggaaagggtgggaggcgggtgagggataaaatactacaaattggggctgcgcgtggtggctcacgcctgtaatcccagcactttgggaggacaaggtgggcggatcacaaggtcaggagctcgagaccatcctggttaacacggtgaaaccccgtctctactaaaaatacaaaaaattagccgagtgtggtggcgggtgcctgtagtcccagctactcaggaggctgaggcaggagaatggcatgaacccgggaggcggagcttgcagtgagccgagattgcacccctgcactcctgcctgggtgacagagtgagacttgtctcaaaaaaaaaaaaaactaaaaattgggtacagtgtatactgctcgggtgatgggtacacccaaatctcacaaatcaccactgaaaaacttactcatgtaaccaaacaccacctgttcccccaaaaccaacagaaattttaaaaaatttaatttaatttaaaagaaatcaatatatgaaaaaagaaaaaaaaaaaaaaaaaaaagaagtgccagtcgggacagacagagaactctcaggaaaactgctcattttgccaatacatcaaatagttatttaaaaaaaaaacaaaacattttctaaagtgtgttagagggctagtgaagagagaaggccatcgaaaatgatgaagaataaggaggagagatgtacaggcaacacaaccaaggagaaaaggaggatgccagacatgggtcaatcttgttagctaagtaaacctcaatggtatctgcctctaagctctgtttggtgagtctctgggacccaactaatgatggtttagtgtcctttaaagaagaatttaaaataatccagtacataggatttcttattgtgcaactttccaattctgaaggaagctatagggcaactaatgttaactaaactgctatgtctccctgttgggtttgcaaagccactcagtactgtgtgatcagtaacccaggaacaaagagggcagtcacacagtaacatcaacacccactgggtacacagagttgcccacttttcatgactcttccacgtgtaagggtcacaaacttgggaagctggtggctgtgttattacccatttagaaacggggaaacagaggattagagggaattatcatcttgaacatctcatatttttaaaaaggaactctaataactacctgacaaattggtgagtgaagagtcttagccaaacactcaatgacaatagtttgaggaagaagcaaagtgtagtagttagaatggtgatttctgagcaagaagatgggggctctgtattcctggccaagtagcttggcttctctgggtctcagtttgctgccaaagcaaacgaggataatactgatcctacctgtaataggaccattgaaaggatttcacaggatgaggtttatgaaaatactttatagttaataattctacatcatatacctgaaatttgctaagagagaaaaatcttaaaacgttctcaccacaaaagataactatgtgaggtgatacatacgctaattagcttgattgtggtaatcctttcacaatgtatacatataccaaaacatcatattgcacactgtgaatatatacaatttatttgtcaattatacctcaatacagctggaaatacataaattttcatgcactgtgtaaatatgagagatttatttctccaacaatgatagaatctgaaagtggggattttcatgtcttatctttgcaatctgaacacagcaactttggatgtcttagccacattgcacggtagactgctacagtaagtttgtttaagtgctaatgcttagaagtcgggcaggcagctggaaccaccatgctggaaaagatacttcctgaaccacttgttcaaatgctttgtaaacaaaagggactaaagagatcccatttattatgttcactgtttaactttggtttctcatctgtactagaaggtcgtatttctgtcctcaaaccattaaaactctatcaggttcccccctccccccaagaaatgctgattttgccaaataagggcattttaaagccttccatctactataacaatgatttcttattttaagttttttttaagaattaaggaataactgacatacgataaactgcacatattcaaattgtataatttgataagttttgacatatatacacccatgaaaccatcaacacaagacagaaattatccaccagcccggaagttttctcgggcctttttgtaacccctttcttgccacccccatctcccctaccccaggtaaccactgatctgctttcacattttccagaattctgtatacatggaatcatatgatatgactctcatgggttagggtcatccatgttattgaaggtatcaatagttcattccttcttattattgagtagtatccatcatacagatacaccacaatttgtttatccatttacctgttgatagacattaggattgtttccagcttttagctattactaataaaactactatgcatattcacgtacgagtcttcaggtgagcacatgctttcttttctctgggagtgaaacagctgaatcatatgataggtgtatgtttgacatgtttgtatcattttacatgagagttctaaatcctacacatccttaccaacagttggcatggctggcttcttaaattttagccattcagataggtgtgtagcagtacctcactgtggttttgacttgtgtttcactaatgacattgaaaagattttttcttgtgcttatctgccatttgcgtatcttctgtggtgaagtgtctgttcaaatcgtttacccatttttaaattttgttttcttattattgaaaatgccatcagttttaatgagtggagcaagactggtaactgagaactgcaacaaaattttacaattcatgatacccaagaggataaaaaaattcacaaagattattttccaaaacttgtgtggagcgaaaatattctccaaatgttatgacaaatctgaacttcttttaaagcttgaaaaggatttaatgatattttatcagtattgctgctaagtctgcacaggttcagactattagtaaaccaaataagcatatttcgatgtactctatcggtacccaaaccatcttaacctctccttcgtgcattagttcaattacccaagcatctatccctaagccacatttcacactttgcactaattatactctaatcccatagattccattttactaattatttcttatgtcaaatttgtgcccacattcaaaaggtgatgaaggccaaaacctctatcgcatttttttatgtcaacagtaacagataaaatgtgatctacaagcatgaagatgaattctcctttccgatccatagagaatgctagatttgagggcacctacaggctttgaggaaaagcaggccccattcggttgtgtagagccatcggttcgtagctcaattgttacagttgatgtgggtttccttttagatgtctggaaaatgactctgctgaccacatccacattctgaaatactttttgagaacttgtaaccaaactgcaggaactgactcattttgcagtgcccagccaccacacaattgttccagaacagactcaagtcaaagggaaaaatatgaaggtcttagaacacagacagcaagttgtctacttatatggggggacaaccgggggaaatcccagagcacatggggcaaaacggctcaagccccggaccaatcttagaggaaggaccaaacagaactcaccacttcgtggacaacacatgtgttttcctcaaagcaagggggtcagaggctggtagaaaaagaaacttaatgtctatctcttagacactaatctacacttagaaagtagattcagtagagaaatgtctgcagaagactcgggttagatgttgtcttgaaagtccattcctgaattccttgtactcccagctcctctgagatgggatgctcagtaagtcaggagtatgccccttgtcttacaggagataagccagcagggacagcatgtccaagatgctaggcagaactgaggctgacacttgagcttaggaccagaaattctctggctcccctggggcttctgtacatcctctcctggtccatttttacatctttctcttaattcccaatgtgtctcacccaagggggtcagtttccccatgatgtcccaaatctttctccctctctcaatgcagacttcttacctaaggggaggatgaagaggagcaaactaagctctcctccacacaacactctatgttcccaaattactcatttctctaccccacaagtgaaactgatttagtcagtcagtttcagccaaaggcggtgaggaaatccggtcttgttgaactaaactataaatgacaaaaccaataataactcttttctgcaggtgggtcccttgctaaaagaatatgagggttaacccaacccaaatctatcattgactaatagaaaggctatgtgataagaattaggtatagagtctcaggcagtatttcaagtaagataaacctggacgacacctataaaaggctatcaagcccctttctaagccctgtatgttgtcgatataattacatatacattttatgtctgttctcacccgtgcaatgtctcttaacatgtaaactcccagatgacagaacttgcccatttccttagatttagtaaggggcatttagtatccgagtataatagtgaagtaatgacagggggctgcaatcaaattatggcaatcaactctacctttaagaaattacaaaaatgtttttaacacaactttacaagagaaaaggtacataaaacaattttacccttcccacctggccaattgcctttatttttccacactctctttgtacctccaataaaataagtactgtataacaagacttcttaacctgtaccaaacagtaagttttcatacagaattttaaaaaggagcttatcatctgactgaacataaaactaagaattattttaaaatgaaagcactttaaacatggatttaaaatcccttcagttcaaaattctaaactgcttgttactgagtgcaaaaatcagcaaagatatgccttatggaagatgagtttttggcaaatttaaatcaaatcaaaacattccacagttagacattcaggtaccccacatctctctgaggagtagatgtgataggaagaattgcccactttgcgctttttagctgtaattgtgcttcaaatagttcaactttatctatctttgctaaggttttcatagcataataatttaaattacaaaagtagcattttactgcaagaaggccttacacggcttgtaaacactccagttatgaggcacaaggggctcgactctccgggatccctacaataaatcacatagactctcagaataccatcttcactctctctagttatcatttcctaccttccaaacagcttcttactgtggccaacagagtcctacctgatctgccatgatgtgtctcttggacacacaaagcctgctcccgtctctactgcagttacttttttattttctctgcctggaatcctcttcctccagacactcccacagctgattcctcactggcctaataacatcaaagaggccttcctattagccctggttaacgtcgctctacccctgatccccaggtactctctctctgacacagctttatttttctccgcagtgtttactaacacctgccgtatacttatgagttccatcaccatcagcctacccgctccatgtgagcggggactttattcactgctgtattaccagacccagaactctctaaggcacatggtagacatggtagatgtataatatatttttgtaaaatgtacatttcccatgtggtgtcttagtctgttgtgctgctataagcttatgaaatttagttggcacctgagacaatttttgttaacaccttaccaaaactccaaacgcctcaagggccaggtggacaagagctgtaggaaagtgatcactcccccagcagtaaaaaaagaaagcaggaaaaagaacagtttctctataatctccctgctacccatgcatagcaaataagggaaggtcttttggagtatggatgtcaaacggaatggggagaaaggtagatattcactgtcattatcaacctaacttgtcctgaggcctccttattggttttaacacagagagagagaagagccttgaaatactgagacattcttttagagtgtgagtgattttgtttttgtttttaaatctacttcaacattttcttcccttgggccatatatacccactaataatgtagacttcacatttcatgctgaaagacaaagcattttcattgcctttgctggtatggtcaaacttgtttcagaaaatgcacaggtatagtttgtgccattgaagacaacttgaagagtgatgtctttcaaaaactataggaggtgatatcaagatttaaataacaagtaaagataatgactctgtcttaaggaagcgtattcctaactgcaacatggagacgagtaatattttttgaaagaatagtagtataaattccaaaagccctcccctatgttcattcctcattttctatatatttacttagagatattttcaaaaagtcataataaatttgattgagggcatggcaacacttcttacctttaaattaattaaaattctattttaaaattatttttgaagacatctttgtgatggcctttgttgtctcttaatgttcttttattataagcgtaggcaggtgaagcagcaggagtagagaaagaacaaagcaatctgtaactggttgtgatcattaattgtaaacgctactgcacttaatatctttaaacaaggaaattatttgaaagcatgagtgctcttagattatatttactgatacgttccctactatgaacccttcttccgccaacattaaaaagaaagaaagaaaaaccatttctctgcactgtttttccctcacaagcattttctcctctcactttaaaaaaagaaatgcagctcccaaaggaagatgcttaaagaccttcatgagtgttgtgagtgtctgtctgtgaaatatacgttgtctccaaagggacaaacaatcagatacaagatgcagtcagtgaggtgaaaggaacatagagtgagtttattgcttctcctctcccgtcccctgatggactctcactcccatcctttctttcacctatttgcaggtagatgttgaatgacttatgcgagagtatggacaaatgaaggaatgaacaaacaaaggaaagaatgaaggccggcatgattaataaatcctccaagagcaggctcagtccaaggccaggggatttttttttttttttaaagagacttccaagcactctgaacccacgggctaggataacatgccctcatcttctaagtcaaaattctcaatctacatcagaaagaggaaattctcaatgtgaaacccctttcccatattctgaaaattaagtccacacccaaacataaggttttatgcacatagatggcttcctgtacttctttatctagaagttttaccccatcctccagaaaatatccagaactagatggagataaagaagaaaaatattagtaaatacagattcttacacatttcatttttctatggattagttctataccagcaagaaggaatttccagaaaggttgatgtaagtgcatccctaggactcaaatgctaacatacttctccctcccacccccactttcaagtgaaaacattagagaaaaaaataggggaagttacatgattaaacttgttagtatatgagatcaactgaaaacaaggaattcccctcctggactgcagtggcctaattaaaactcataaaacacaaatgactaagactgttcccgttgatttgtgaaataaaaagcagaaaaagttaattttgtatttcaatattgacagaggtaggcctagaagacgtgacactttacagaatagaaatgagaagaccatttccgagactttcaggttcagtcaacttttattctgctttcctgccagaagtacatgtacttaccatctgtactggcaacagcctatttggatttagattctggttccatgacagatgagtggccctaagtaagttcctttacctctctgtgcctctgtgtgttcatctatgaaatgggcatgataattgcaccaatagtttgtcatgaggaaaaatgggtcgatgcaggtagagcccttacaacagtgcctgtccagaacatggtaactgcacaataagcgacagtcaccatcatcagtgttttgcttaatctgatgtgaaaaaaagtcatatcacttagcatggatctacaggctttaggactaaactgaagaagtctgttcctaaagggattttggaagggaatgcaagtgtgttaagcaccattactccaggtcccacagcatgtgctttacatgtgttatctcacacaacaaacctgtgcactacttctgatgctctacactctggggctcagggaaatagcggagtagcttactcagctagcaaggggcaaagggagcttaaagcacaaatctacttatttccaaagcctgggcctcttagggagtaaactacttcaatggaggctgtgaatggacaccctcttggggtcatgggtaccactttcacgcactaacactctctggaaaatgtctgaagctttcaagatttttttcaggtaatccgaactctgaatgttccctgcaaagttttgccgggcgtgtacatatttactgtttctctcaactttaagaactctagtctcacttcagatatattatacaaatcctaatcaagaaaaaaaaaaatcaatggattttcacttttaaaaatctttcttccctctccttttaggaaacgcagaaaaactaagctttctttcaataccaacaccaacaatgggctttcaataccataagcacatcaggggaattaaactcttccatggcagaaagaggagataatttaaaatgaaacctcagcctactcttcatagtctaccttaaatagttatactatgtttttaaaaagcaagttattactttagtaaccatttaaaagaaagtaactagaactattttgttataaagcatagctaagaaaacaaaatgtcccaatcattatattaacttacaaaagcatactaaattcaacttttgtatgtatctaatctgttcctttaagaattagtctaggccaggcgcggtggctcacacctgtaatcctagcactttgggaggctgaggcgggcagatcacaaggtcaggagttcaagaccagcctggccaacatagtgaaaccccgtctctactaaaaataaaaaataaataaataaaaaataaaaaaaaattagccgggcgtggcagtgtgtgcctgtaatcccagctactcgggaggctgaggcaggagaatcacgtgaacccaggaggtggaggtttcagtgagccaaggtcacaccattgcactccaggccgggtgacagtgcaagactctgtctcaaaaaaaaaaaaaaaaaaaaaaaaaagagagagaaaagaaaagaaaaaaagaactaggctaaagaaaaaagatcaactaaaatgatgcatttacataaccacattgtttatagttaataatatatgtgggggtttttttactttatgttttagattgccctaaatatgttggaaagaataaactagaataaatatggggttgaaaaacaagaggttagagttgaggattttaagaacttgagtcaggaaatattcaaggttaaatcacttacagtctttaatgtgtagaataactgtttaataattgatttatttttcaaatgaaaacagtaggaagtaggtaggtttaacaggtcttactcccaaaacatgtcatatacagttacccagttgtctatttaaattgaaggtagttcataaaatgcaagtgtttactttgcatgttctccttagtaacttaatcttctggatttgttacccaatgattatattcaaacttggctcaatttcccctcctgaatgaagacgtctattctccaaattcagactgtataaccagtacagcttgtttaagaaaaataaatatgataactaatagtaaaaaaaaaaaaaaaaggcaaaaaatcatttatttacagcagtctgagattgataggagggaatgagttagaagatgagcatcaaaaagaaataaatctaggacctttaaatgtattcaaagaaaacaatactgctagtgtctaattaaaatgtcaaatgaataaataagtaagacatacaatatgtcagacagaggcaagtgctaagaagaaaaattaagcaggaagaaggatagaaagctggggaatagaatggggaggttgccatcagtttgaaatgaatttttttatccctagaaacatatagggacttgagacatgccttatatacattttttgagaagtactgttaaaggtatccttttgtgaattcaaagagtcatgcagctgaagctccatgggctgcctgatttctgccaagaggctctgctgtgtcccagtgtagttcccaagccagggagctcacaaccttggaggtgacccatgccctctttattgattccacacctcctgctgggtaaggggtctaaggaatgtctacaaaaacgtttttcccactgttcaaggaaacttccttagggttaaggaaagagttatttcctatgtcttaatttttcaagatgaaaaagtcgggctgatttactgatggagatcaccttgggaagcctgtgaggagagttcagacccctggaattcctacactcccacccaggagaacctgttataagcattcaaccacagccccggctaatgaccatagtggtgataccaccagctcttgatcgtaggaggtatagggtgactatgaataaagtaaatcactcaaacaccccctctgactcagttaagaagtccagtgccacatctccagtcctctcttgtacctgcatcagaatcattaagagcagattggagctagactgtctgctttcaaatcttggctccgctacttcctgtatactgtttttgtgagttaaagaatttaataagtgtaaagcagttcctaccaaaacgtgtctactaagtacctactatgtgccagacactgttcttagatgccagtgattcatttagaatggtacccggcatataatatgaactcaatgtatgtcagtaattatgggtccacaaatgcttacctgacactcagattgattattattattattttataaaggtaataggttgactattcaatatagtatataaacctctaggggagtctggaacaatactccgtgatcaaacacattaatacttctacagtaaaacatacaaagattcattctgagcgagctaaacaaagactatcattagcttcacatcagttcaggtcaggatttgctgccaaatttgttacatgaaaatcttttgattttcagagctttttggattacagaagagatggtgggcatatatttattaagagactaaccccactgaaatctttttctttctaacttcaggaggttctagcaaccaaataaatagttaaaactatttaggagtaggaaataggaagaccttcagacatggaaaatcaacaactgcataattaagctatgccaaatattagtctgaacaatccctctcctcaaatacagtgctccatagattctccattgacagacatttccacaaacaacaggtctcaaacaatctttttctaagtacttttcaaaagcactttttgaatatagaataaaatacttaaattttatcactattttaatagtacaaccttgtctttcccatagaaaaaagacaaaagctattaaatgacaaatgaacaactggtttaaaaacatgtgccttaaaagaacacagtatcctctgtagtctgcctgggggagatgaataaacgttatgccaaagtggtaaaccatcctgctaccaaaggaattttctccacattgcattttaaggaaattcacagctcttgaagagctatacaataactggttcaagatgttctcactgctggtcagcactggataaaggatttgcagaaacccatggaagcctatttctcttgcctctttattgcccccatgtgttgttatttatcttccccaacttttctgaccctttccatgtatttttttaattgaagtattgctttgttcaagacctatgtttaccactcccatggcgatcctgtacacaaagacaagtcaggaagacatgaaacgaacggagatacttatgttgcttcatggtttttccccttctcattatcctcctactcaatgagactatagtgggaggtctgaatgacatttccaaaccaagaacttaaagctacatttcaacacccaactactcagttgtcataggaacaacactatgaggcttatctgggttctaacaaacagccacttgtttcactaatgattaaaactcccccttcaaatcaaatatagacacccatacatatacagacctcaaaagaaaaatttaattgggtaaaactgtatactacaccaaaaacttaagaaacaagcccaaagggaaagcatttacgttcccgaacatgcaaattcaaacactatttcagagaaattattttgaggtctgtctcttgaccagatcccttcagtttgttgttttacacacccacaaagacaaaggcatatgcatggcattaatatcttttaacagggtatacgaaaatgtgaatactctcaatgaccccagaggagaattcagagcaagcaatgctactcactttcgatgtacttttaaaaattaacaaattgagaacagagaacggcaaatagaattgaaaacatgaagttctcagttaattcttctgggatatactttctagcatttactgttccaacctgtttctatcacattttgtcattcaaaacaatggattttaaatggatgaggaaaacctaaaaattagaggcttttttccaacaggcacggcagtatttatccagattattaaatcatcatgttctccccaagtatttacttacatgaaatacagagttgaaaacataagctagcagttgaatataaattatctgtaaataccttaatgctttgttgccatttttctgtcttcaagactctaaaaacctataaattcatgtgcttcaagaaaactaatgccattccttaattaagtcaaattgacttgtcatgttcacaagtttggatcacccgtttcctgacttattggaggacctgcccttaagagccgtgcttatcttgtctttctatttctttaagaataaatacttatgcaaaagtcttgagagctgctagtctgagaaaactgatctcaaaagttatccaagtatacaagagggggaaaaaacaattaatatatctcactagattcatctccctcccccaccctcatcccactccactgctaagagagagaaatttcagcactgctatcctgttttattatacattttcccttttgagttaaggattttaagattttgaaagtaacagaacaggaaccaaaagtagattcaacttccaatttggcttaaaaagaaagaaataattattatttcctatattacccaaaacttattctgttaataacagttataattatatattcaaattaataaatgaagattgctaaaattgcctatatacttgttagcagttaaagaagaaaaattttttccatttgcttctataagtagacatcacatgattacttctattgaccaataagaaactagtaaaatcaggcagtcacccaccattcttttctaatgttctttttcttattctattcaaccttttcagtatattcttaagaagccaaatcaagaaattagacattcatgcctaaaataaaattgcgttaccttatacatcatgaacaggaacctgttgtatataacacgggtattcaaagctttattgtctttttctagaaccctttaacataaaggcagctcagattcaagattagaaaactgaattcaacaggcaggaacacgcatacgaaaccagtaagaactactaatcacgacctctcaaaatgtcatgaaccatatagatagaaataaccccccttttgctgtactaatgtaatccaatagaacaaacttaaaattcgtgacacaaatgtaagaaacaaaaaacaaaaatctattgccattgtaatctacccttcccaatcaggagaggtgtttccgacgcattacttgaactttcattttgtacaactttcatcttgtaaggttctaactaaatacttgacatcttaatgcagaggaaaggaaaggagggcaagtagactaattctgaaagcatcccttcaaatttcatacatgctattcagactaaatggaaatctacatccatggaaagttaatgtcgcaattctactaaacagcccattctgattttatgtttctcctccactaacaagaaaaaataaaacaaccaaatctagctgtattacatatgtttagctaaactgatagcactcagctcatttttgttaattacctggcttcttctcagtctttatgcggtattctcgtgctgctcttttttagaactcctcactgtttatgtgttctctgttcaacacagttgttaggggtctgtgaacaatttttcaattcccacacacgcatatgatatctattagggagcaatgccacttttcacttaccaattctggataaaggagtatttcctggtgacagaatgctgctgcttccgttcactaaaactccctcttcgcagcttgataaatctgattataaaacgtctttgttccagatcacacgaggcgcttttcctacaaaagttttctaaagagttatctgcatttcattccagttcaggaagcctagagtttgatcaagtcggtcacaaccactttgagagtcttccactggtgtgcggactccaagaaagcagtcacttggtcatctatcacatgtggctgaatcactggacagaccacccccgccccacacacccccagcccccgttgagcagcagcccaggcaggagagt

SEQ ID NO: 18745 - RNA, 11382 nt, Homo sapiens
  source 1..11382: mol_type = other RNA
tgagtgtgtgtgtgtgagtgtgtgtgtgtgtgtgtgtgtttgcataagttacagttattctgggcatcaaagtttttccttaaaaaacctaacaatgcctaacttgagtgattcacagacttataagaaaattgaaaccatgtatatgttagaatgttatctaacttaaaattacatatctgtggaaaaactttattgtgatacttttatattaaaaatcagtcacttagaagaaaatatcaaactttaattacaatgatactcattttctgtaccgagttgtcaggaggtataagctggaaaccaggatggcgccaccatcacagctgagaatgatgacaacagaagtcttcattgtagtgtgtcaggtcttttgaggtaccaagaattgcggaaattattttcttctatgtatcttactctgtgataattttttcttattttttaaaaatacagcaaaacacacaataaaacacagcaatatactgaggtctcacattctcacggcttgtcttcctacacttattccaattcagagtacactttgtatacatctcttcgctggttagttctgaaacagtactctttcttatatttgttttaaacatctccaatactgaatattgtaggagtctatttgcctgaaagatagcacttgagctgaacgaaaataatctattcagtttggacatacatcctgaccccaggttttatgcttcatgtctcatttccaaggttaaatgaactggattttcaggatcaattctgcagtcaattgaattaacatttttaaggctcttttactatagaagtgactcttacataagcaaaaatattataaaagtggttttctttttaatgtaattataatggaatctcataaacataaaaattatagtttcattgaaagtaatgctgtgtgttttactaatgtgaattgttcgttcctctaaatttgagaaaaaaaattctgaaatctctactaaagagaaactttacaaatgtgcaattctccctcagtatgctcatataatttaattgtagaggttggatctaatagacatcttaaaagctaaaaagaaaatatttaaaagtcatttactttacttcaacatttcgcctcaaattgtgtgtgttcctgcacacgtgtatgtatgtgtgcgcatgctgtctatatatacacacacacatacgcacacaaaattcaaagacaaatacataatatatataagttgtgtagtgacttatttttccttttccttttatttttgggcatttaaaattactgcatgtaaaatgaaattgctatatagttacacaggaaggggaacaccacactctagggactgttgtggggtagggggaggggggagggatagaattaggagatatacctaatgctaaatgacgagttaatgggtgccgcacaccagcatggcacatgtatacatatgtaactaacctgcacattgtgcacatgtaccctaaaacttaaagtataataataataataaaaaaacttgattgttcttaaagtattggtcatatacagtatacaacatattccagatcttgatatacaaaaacatagggtttatactcacaaaattagaacatgaagctgtagggtagtgaatcatataagtttttcctgcttatataaaccattaacatcattatattcattaataaaatgaaaatgcaagtttgtttttgaatgaaagtatgctgtactttcaacattctcattagttacatagttattaatatatttgtttctagtgtctgttcacatgagcataaaataaccagataactaagagctaaagttgagaagagagcttattaacattcatcttggcatcactgacaaaaagtaatatccattatatattattttttagtttcctagagtttcttcattcgtaagagattaagatgagctgttgtaagatataagtgagtttgagtcatcaagagtgcattgcattcaggatggttttcatgttaagtcaatatcattgcatctaattttttcaagtgtataaattattaattacacatatgtcactgtgactttaaaaagtattgtattctctagaacttcattttctttatctactctggatgcctggaagaccacttaacttatactcattattgtctttttctctattctggtgttttgtgttcatcaatgaggctgggatcatctaaaggcagtcctttatcttccactcagttatcattataagtaagaaagatttgttctttatttataatcccattcacatatggatatcattaattcatatgaatggttgaattatgttgagttaaactgcaatcttctgagatcttataaataactgtatttgagtggcttcaattaattatgacaattatctatttgaatattattttccaatttaggataccaagttgcatatatttttccttaatgtatgtatctccaaacagaaattctctgtttaccatataacaattatcaacctttttatataattcccattatttcccataataaagctttatctttttatagtgttttactgtttacacagtctttcacttaatcattcacaagcctctgaaacacaatagtaattaactcaattttaatcatgaagctataaaagttcagagaatgaaaatggcatctagggcacagcaaaaatgtggcgaaactgagcttctgacctagattttataaccacagaccagaggtaatttctggtataccacactgacaccaaagcccagtaacatttaataacaaataattcacactctatattctgttaacaatgagattaaatctgcacaataatatgtgacaattacacaaataacagctaaatgttctttccttagccaccaaaatccttaccttaatataaattagattgttacagcaaataagatatttctcctttcattcggtaccatattttctagtcttattgcctaacagtcacttggcaggtgacaacaatacgccagcattaaccaggaattatgagactcttatttttacattacttcagatacatctctcaaggttcccaatcacacacatgaaaacgcacacacagggccgggcgcggtggctcacgcctgtaatcccagcactttgggaggccgaggcgggcgaatcacgaggtcaggagatcgagaccacggtgaaaccccgtctgtactaaaaatacaaaaaaattagcggggcgcggtggcgggcgcctgtagtcccagctactccggaggttgaggcaggagaacggtgtgaaccctggaggcggagcttgcagtgagccgagatcgcaccactgcactccagcctgggcgacagagcgagactccacgtcaaaaaaaaaaaaaaaaaaaaaaacacaggcacacatccttttcagttacattctaagccagtagaagttagcataacaatgaaaaagtgtcagaatgcaacgcacactgcctgtcttgatttgcttgaaaaatttcccacagaattatacgttacaatgtcggccaaatcacagccttaaacatctcccatttttcttaagggcttatcccactcttctgaaatagtttcaattacatttaaaatgcaaatgctattattcctttcttgttctttattatatccagccgactaacatgattgtattagctttcattgccaactttcatacaccgtcatatatacacacaatatacattattaataattaaaaaataaacatacactaacagaaaataaattggtttatctattatttgtcatatatatttcacttgcctccaggcatcgtggaccagaaagagttaaaaaataagttgaagctttcatcaacttcaattggattaggtcaactgtaaataaaactttaaatggtgacttggaaaataattagtgttattattagaacagtttgtaagtgaatacatgttaaattgaaaatctgaagattaatatttacagctagtgctttaaaactttaacatgtttaaatcatttagcttcttgcagtttgtttagcttagcttattttaagctgctttagattttatatttcaatataaatgctaacaacactatttgcatttgcatttcttgggcatgtggatcacttcacaaatatcattcctacattgtgtaactatgccgttgacatgaaaataattgcctatgtctaccatccaatgtagtaaatgtaattgtgcatgaagataaaataatttaaaacttcctcagagggcagagtgaaaaggcagctaccattacttaaccactactacctcctgcatgtatcttgtagacaactaacctcaattgtagtcatcagcagagcttcctggcaaataaagacatttaccagatcccagatctggtgattgcttgtagaaaaatcaaaaatctacttattgcctgcaaattactacctaattttttattgatgtctctttcctgattttgttccttagctggctgatcttggaatatttctttcagagactaatttgtgaattgagattgataatttaggcttgatctccagaaatccatttccttaagatttgatttttatatttttatgttgatttttaataatgcaatggtgacaattcagattaagggcttgggtgtatttccttgacatagacagtaagaagtaaaatgcatctgatttttcaataaattaaactgttcaaaatgggcataatttggcaaaccctgagtttctattgatgctcctgtatggacaagtggaaaataattaaatatattgacttcctgaactattatctctacttgaaatttagccattgttttccataaagaagtgactcctctccctgtctacaagtagctccaaggatttcacttcaggaaatcactaccacatacattgttatttagtagtaaaatatagcataaattcctttcatgtcattattttaaatcatataaattcatactatatttacaattatgacatttcattttataaaataatttaagcagtagagtgctggtaaatgtttaacaacttgttctccagagaaaagggtagtgtttgctgattactgttgtggtctaaataatcccaccaaggctgacatcaacctaccaaaatgatatcactgtacctggagttgggaagagatatgaagaattagttcctgtgagctcattctagttggtttcagtataatactgaatttaagcaacttgataatatatatttatttaaatcatatttggagaattttccaactagacttaatattaattttatcaatcagctcttcaatcactgtttttaaaacaaagcctatatctcaagtattgacagtcatcatatatagcattagatttcagaagaaaaaagaaaactaaaataagcaacggcaaaaaatttactactattacaattaagcttagaatacttcatataaatactacctatattaggaacattcttccagccatctcaaaaattaattttttaaattaatttttttaattaaaaaataccactgaatgaaatgtaatactgtattcatataatcatccacacataaatagcaattgggtatatgcaataattttaaattattatttaaacatgaacctttctttttccaatctatcattggtaaccatttgaaaaaattaatgagaaaaaacacacattttaaaagcagaaaaagcagggtgaatgatgtgtgttccttttctaaaatacatccacacctccgtttagtggtatgtgcaacaatcagcagttttgacatcatccaaatgtactaaactatttcatcttcttgcagacaacaaggggattattacaaactgttttctcagcaccttgctgacttaacaactctgtaattcctgcaccacactctgattttattgaactgggtaaatacgcgtgtttttttgtttgtttgttattttttagtttgaaaaacttgcatgtgtgattaaaagttatgaacagtatctttcactgttataattttttaaaatatatatgcatattaatacagcaagaagcatatctatatagtcataaaacaatgtctacaaaactctattcaaattaaagaactgtttgcaggtaatgaaatttattggattatttatacttatgaagttgaaggccacttttacatacttcatttctaaagttgggctgcaagtttacagaatcctacatagttcttctttgtgtaatcaacatattaatattctaattccactgtctacctttcaaaaagcacttttagaacatgattctctacacagtgtttactatctgtaaatgtattaggaacccaacaatgaattatttttaaaaggagaaaggaaggaaaaaataaatccattcttacttgaatgtatatgcacattaaactagtattaatctaggaaaaataataggtagaaacatcattttggtcatgaaagtcatactctaacaagctcaactcaaacttaaacacatgatgacttgcaattgccttccttcctttggcacatctaaaccacacagaaatcatacattgcttggttaattcttgagggacatatttgcatcagaatttaaagatggattttaatttttataacattatattaagacttttaaaaactcaatattttactcaataggtttgcagcaagaaaggttgtgttcttgaaatcgtctttggagcatgtagaactcatgatcttgaaaaataattcttgcatcaaagaaaatctcaattctctctgaagtctttctaaaatacaaatattttattccaatgttttgacattctaatggctcagaagaacaatttatatgtccttgtagctgtgctcctctttgagatgtgacctgcaacagggctcaattgctttactattagttctccatttccatgcttcatttccttcatgtagctcgggctggagaaaaatcagcatgttctgatgagtttaatactatgaggcagtatgatggacctgaatttagtggagattggagctccaaaataaatacaacaccatgtgtcaaataaaaaagaaaagatattctcctgtacaaatcagaagagataataaaaatcaatgaacagacagcaacttttttttttatcatacctacacaagcatctcaaaactatcaaattatttacctttttcttatttggaacacttcataatttattggataaacaatggtttatattgccttaaactaaattttactggcttttgtggtagggttttcagttaggaaggaatttctgggaatttatatattcctaaataaaatatttctgttaatcaagagcaacataattctgttggattctataatatagtaagctataagcatctctgtaaattaaatttgtcccaagttttgatatgcaacaagttccagggtttttcaatagctcatcatgttctattcctctcaatgacagtaccatgaaggtatgtacagggcatctttgactcactgacaacacagggcactactttctcatagaggtttggtgcctttgcaggtatatgagagttgctatctattcacaaaccactgagcatttatttttatcaaaaaaccttcaaatgctcagagtctgtggtcagtgcagtcctttagataagtctaatgaagatatgcctcaccaaggcagaaatctaaacaattaaaaatggagaaatatttacaaccatctgtctccagcaaggggagttcttgttttctgtatgtagtggtttattattttatttcattttattttattttttgctgttactttttcttcagtacatttcgaattaaggttccaaggctatgagtacaaactctcttggccagtcccatacatgtccgcgagtcgtttaaagcgaggtccccagtcacttaggtagtcatagttctgatcagagtttgagctgatggaatctaaagagctgagtgattcagcaactgagccatttccttcaaaagcatatgtctgcagggagtcataaggaggagcaccaggatcaacatcggcttcttttaatctttcccaaataaattccctaaagatgacattatctgggatgcttttaaaagctggtcgactcaggaattgaatttctggagtcacatccctccgggtcttggtgtctcggatgacgttgaggtttctcagtgcagccatgtcaaacgcttccgtgtcctcctctcccccgccctcgtcatcgtatctcacaatattttctctgatgtctctttcttcgtcaaaaataaggggctcttttttccgtcttctcatagtgacgataaggaggatcaacaccaataatgtcaagacacaggcgagtatggctatcagggctcctgtactgaggccagcaggtaggacataggcctctgcattgcaggtctgggctacgccgtcagcatcacagtcacacacgcggatggtgagggtgttggtgctgctaagtgagggagatccactgtccacaatgaaaattggcagatagtaaactgattgttcctgtctccggaagccgtttctcctggtcagtattgaggctgtgttgtctttgttatctttcaatgaaaagttgtggttatttgttgcatccgttgttaagctgaagtaaaactggtgtccattggatggctcatctttatccacagcactgattttctggataacctgccccggctgggcattttcacagacggtggtctcatagtccatggcaaattcaggggcgttatcattgatgtcaagtatagtgatggccacatagcctcttcctacttgagatggattctggctctccattgcaaggactgtgatattgtgaatagcatttgtctctcgatccaaagacttggcagttgtgatgaccccactgttggcatcaatattgaagtatctctccaagtctgtgtttctgtcaattgagtacctcacagggctattggaagaatctgggtcatgagctgctacagtgccaatgatattcccaacctgggtagcttccgacacctccatagggtacaagggtgaagagaacacagggggctcatctacatcttccacaattatcttcacagttgtcgtgtcactgaacggacccaagctcagaaagcgagggtcggcatctttatttgcagcttctatccgtagcgtgtaacttgttttggcttcaaaatccagctccttctgtatagtaatgattccttcctgggtttctttgtcaacagaaatcttaaaaatgcccaaaccatcaccatccacaatcttgtactccatttcagcattagctccaatatctgcatcagcagctttaattctggccacaactgaggctacaggtaatgactctgggacgttatattgataagaccttcgaggaaagcgaggtggattatcgttgacatcagttagggtcacagtgactgatgtagttcctgacagtcctccattttgaccaaccatatcctttgcctgaatgacaagcaaatactggtctttagcctctctatccatgtttggaagggcagtcttgatgactcctgtctttggctccactgagaagtacggctgtccttgcagaatactgtagaccactctggcactgttgccatatgtaggatcatcagcatccgtcgctgtcacttgtaccactgaggtccccacgggagacatttcgggaactcctgccgtgtatgggccatccaaaaatttgggttcattgtcgttgatatcctgaattttgatgacaaactccgactcgggctccacgggtttgttggtgagcctatccagcgcttgagctcggagcgtgtagtaggcctgctcctcacgatccagtctcttggtggcatgaatatccccagtgttctcatcaataatgaaaatggaacttgccccttcgcctgacaagatgtatttgatggaaccatctcctttatcaacatcagagtgaagctttcctacatagagggggtctgaacccatgtattcctccagcacaaagaactgattccacacccagctgcgcttggtccgggacctccctgattggaaatagggctttgatctggaccttgagagttctgcttgactcatcccagaaaaacacaggaaaagagctattagctgcagaaaatggcagaactccactttgcccaacttcatcttttttttttctttctttttcctgtgtaagaaaaaaaccttgacaagagaaaaggcacagttccagttggcttagtagctcttgcctccggcagggtgtcagctgggagtccagagataataatctgtagagtgttggattggaagaggtcaccactgctgaatagccttcgccaaagaatggtgtagtaagtacctgaactatgacatttaagaaatccgtagggttaacgatctaaaacgtgaagcggtacagaataacgggtcttttctcattaatccacactggaaggttgaataccggcaagtagcagtgtaccatgtgcacccatgaagaagtccaccatgcattcagagaagcagggcgcccttttcccagcgcacacttaaggtactgccaggcggaggggacgcaggatgcagatgaaccagatcagcagaatactaattacaggggaaaaaagcaaagcaccctgaagtgagctccaccttcacgaaaggtaaaaggtgtccagagcgaatggttcaaaggactcctgcccaaagcggcgcatacccccttccagcctcagacctctgcagaacccggcggcacagccggcgcggagttgtgcccccatcagtccgaggttgagggaggagcctgcttgtggtcctctttgaggagagtgctccagcctgcccatgtttgccgctgcacctggagagtgccgggatttgctcttaccctcaactactactcctcgtgtcgcacctggtgtctgtcaacaccggctttccgggccaaacgcccccgcctccgtccacaagcctgtcctgccttgcagagccacatctcactgcaacacgcagtaacttggggacgccaagggaaactccacacggacatccccgcccgctctccgctcactgattagtcctgcttccaaaggcgcacagcaagggcgcacatctgcccagcggcgcctccccagccccgcgcaggcagacacactcacctggggcctcgctgccctccccacggcgtcagacgccagggacccgggcgtgtgcatccgaaagaacgtgcgctcggctgccggacgcccgcgggctcttggggacccagtgcgcgcagctccgcgcgcggggcagact

SEQ ID NO: 18746 - RNA, 10580 nt, Homo sapiens
  source 1..10580: mol_type = other RNA
tgagtgtgtgtgtgtgagtgtgtgtgtgtgtgtgtgtgtttgcataagttacagttattctgggcatcaaagtttttccttaaaaaacctaacaatgcctaacttgagtgattcacagacttataagaaaattgaaaccatgtatatgttagaatgttatctaacttaaaattacatatctgtggaaaaactttattgtgatacttttatattaaaaatcagtcacttagaagaaaatatcaaactttaattacaatgatactcattttctgtaccgagttgtcaggaggtataagctggaaaccaggatggcgccaccatcacagctgagaatgatgacaacagaagtcttcattgtagtgtgtcaggtcttttgaggtaccaagaattgcggaaattattttcttctatgtatcttactctgtgataattttttcttattttttaaaaatacagcaaaacacacaataaaacacagcaatatactgaggtctcacattctcacggcttgtcttcctacacttattccaattcagagtacactttgtatacatctcttcgctggttagttctgaaacagtactctttcttatatttgttttaaacatctccaatactgaatattgtaggagtctatttgcctgaaagatagcacttgagctgaacgaaaataatctattcagtttggacatacatcctgaccccaggttttatgcttcatgtctcatttccaaggttaaatgaactggattttcaggatcaattctgcagtcaattgaattaacatttttaaggctcttttactatagaagtgactcttacataagcaaaaatattataaaagtggttttctttttaatgtaattataatggaatctcataaacataaaaattatagtttcattgaaagtaatgctgtgtgttttactaatgtgaattgttcgttcctctaaatttgagaaaaaaaattctgaaatctctactaaagagaaactttacaaatgtgcaattctccctcagtatgctcatataatttaattgtagaggttggatctaatagacatcttaaaagctaaaaagaaaatatttaaaagtcatttactttacttcaacatttcgcctcaaattgtgtgtgttcctgcacacgtgtatgtatgtgtgcgcatgctgtctatatatacacacacacatacgcacacaaaattcaaagacaaatacataatatatataagttgtgtagtgacttatttttccttttccttttatttttgggcatttaaaattactgcatgtaaaatgaaattgctatatagttacacaggaaggggaacaccacactctagggactgttgtggggtagggggaggggggagggatagaattaggagatatacctaatgctaaatgacgagttaatgggtgccgcacaccagcatggcacatgtatacatatgtaactaacctgcacattgtgcacatgtaccctaaaacttaaagtataataataataataaaaaaacttgattgttcttaaagtattggtcatatacagtatacaacatattccagatcttgatatacaaaaacatagggtttatactcacaaaattagaacatgaagctgtagggtagtgaatcatataagtttttcctgcttatataaaccattaacatcattatattcattaataaaatgaaaatgcaagtttgtttttgaatgaaagtatgctgtactttcaacattctcattagttacatagttattaatatatttgtttctagtgtctgttcacatgagcataaaataaccagataactaagagctaaagttgagaagagagcttattaacattcatcttggcatcactgacaaaaagtaatatccattatatattattttttagtttcctagagtttcttcattcgtaagagattaagatgagctgttgtaagatataagtgagtttgagtcatcaagagtgcattgcattcaggatggttttcatgttaagtcaatatcattgcatctaattttttcaagtgtataaattattaattacacatatgtcactgtgactttaaaaagtattgtattctctagaacttcattttctttatctactctggatgcctggaagaccacttaacttatactcattattgtctttttctctattctggtgttttgtgttcatcaatgaggctgggatcatctaaaggcagtcctttatcttccactcagttatcattataagtaagaaagatttgttctttatttataatcccattcacatatggatatcattaattcatatgaatggttgaattatgttgagttaaactgcaatcttctgagatcttataaataactgtatttgagtggcttcaattaattatgacaattatctatttgaatattattttccaatttaggataccaagttgcatatatttttccttaatgtatgtatctccaaacagaaattctctgtttaccatataacaattatcaacctttttatataattcccattatttcccataataaagctttatctttttatagtgttttactgtttacacagtctttcacttaatcattcacaagcctctgaaacacaatagtaattaactcaattttaatcatgaagctataaaagttcagagaatgaaaatggcatctagggcacagcaaaaatgtggcgaaactgagcttctgacctagattttataaccacagaccagaggtaatttctggtataccacactgacaccaaagcccagtaacatttaataacaaataattcacactctatattctgttaacaatgagattaaatctgcacaataatatgtgacaattacacaaataacagctaaatgttctttccttagccaccaaaatccttaccttaatataaattagattgttacagcaaataagatatttctcctttcattcggtaccatattttctagtcttattgcctaacagtcacttggcaggtgacaacaatacgccagcattaaccaggaattatgagactcttatttttacattacttcagatacatctctcaaggttcccaatcacacacatgaaaacgcacacacagggccgggcgcggtggctcacgcctgtaatcccagcactttgggaggccgaggcgggcgaatcacgaggtcaggagatcgagaccacggtgaaaccccgtctgtactaaaaatacaaaaaaattagcggggcgcggtggcgggcgcctgtagtcccagctactccggaggttgaggcaggagaacggtgtgaaccctggaggcggagcttgcagtgagccgagatcgcaccactgcactccagcctgggcgacagagcgagactccacgtcaaaaaaaaaaaaaaaaaaaaaaacacaggcacacatccttttcagttacattctaagccagtagaagttagcataacaatgaaaaagtgtcagaatgcaacgcacactgcctgtcttgatttgcttgaaaaatttcccacagaattatacgttacaatgtcggccaaatcacagccttaaacatctcccatttttcttaagggcttatcccactcttctgaaatagtttcaattacatttaaaatgcaaatgctattattcctttcttgttctttattatatccagccgactaacatgattgtattagctttcattgccaactttcatacaccgtcatatatacacacaatatacattattaataattaaaaaataaacatacactaacagaaaataaattggtttatctattatttgtcatatatatttcacttgcctccaggcatcgtggaccagaaagagttaaaaaataagttgaagctttcatcaacttcaattggattaggtcaactgtaaataaaactttaaatggtgacttggaaaataattagtgttattattagaacagtttgtaagtgaatacatgttaaattgaaaatctgaagattaatatttacagctagtgctttaaaactttaacatgtttaaatcatttagcttcttgcagtttgtttagcttagcttattttaagctgctttagattttatatttcaatataaatgctaacaacactatttgcatttgcatttcttgggcatgtggatcacttcacaaatatcattcctacattgtgtaactatgccgttgacatgaaaataattgcctatgtctaccatccaatgtagtaaatgtaattgtgcatgaagataaaataatttaaaacttcctcagagggcagagtgaaaaggcagctaccattacttaaccactactacctcctgcatgtatcttgtagacaactaacctcaattgtagtcatcagcagagcttcctggcaaataaagacatttaccagatcccagatctggtgattgcttgtagaaaaatcaaaaatctacttattgcctgcaaattactacctaattttttattgatgtctctttcctgattttgttccttagctggctgatcttggaatatttctttcagagactaatttgtgaattgagattgataatttaggcttgatctccagaaatccatttccttaagatttgatttttatatttttatgttgatttttaataatgcaatggtgacaattcagattaagggcttgggtgtatttccttgacatagacagtaagaagtaaaatgcatctgatttttcaataaattaaactgttcaaaatgggcataatttggcaaaccctgagtttctattgatgctcctgtatggacaagtggaaaataattaaatatattgacttcctgaactattatctctacttgaaatttagccattgttttccataaagaagtgactcctctccctgtctacaagtagctccaaggatttcacttcaggaaatcactaccacatacattgttatttagtagtaaaatatagcataaattcctttcatgtcattattttaaatcatataaattcatactatatttacaattatgacatttcattttataaaataatttaagcagtagagtgctggtaaatgtttaacaacttgttctccagagaaaagggtagtgtttgctgattactgttgtggtctaaataatcccaccaaggctgacatcaacctaccaaaatgatatcactgtacctggagttgggaagagatatgaagaattagttcctgtgagctcattctagttggtttcagtataatactgaatttaagcaacttgataatatatatttatttaaatcatatttggagaattttccaactagacttaatattaattttatcaatcagctcttcaatcactgtttttaaaacaaagcctatatctcaagtattgacagtcatcatatatagcattagatttcagaagaaaaaagaaaactaaaataagcaacggcaaaaaatttactactattacaattaagcttagaatacttcatataaatactacctatattaggaacattcttccagccatctcaaaaattaattttttaaattaatttttttaattaaaaaataccactgaatgaaatgtaatactgtattcatataatcatccacacataaatagcaattgggtatatgcaataattttaaattattatttaaacatgaacctttctttttccaatctatcattggtaaccatttgaaaaaattaatgagaaaaaacacacattttaaaagcagaaaaagcagggtgaatgatgtgtgttccttttctaaaatacatccacacctccgtttagtggtatgtgcaacaatcagcagttttgacatcatccaaatgtactaaactatttcatcttcttgcagacaacaaggggattattacaaactgttttctcagcaccttgctgacttaacaactctgtaattcctgcaccacactctgattttattgaactgggtaaatacgcgtgtttttttgtttgtttgttattttttagtttgaaaaacttgcatgtgtgattaaaagttatgaacagtatctttcactgttataattttttaaaatatatatgcatattaatacagcaagaagcatatctatatagtcataaaacaatgtctacaaaactctattcaaattaaagaactgtttgcaggtaatgaaatttattggattatttatacttatgaagttgaaggccacttttacatacttcatttctaaagttgggctgcaagtttacagaatcctacatagttcttctttgtgtaatcaacatattaatattctaattccactgtctacctttcaaaaagcacttttagaacatgattctctacacagtgtttactatctgtaaatgtattaggaacccaacaatgaattatttttaaaaggagaaaggaaggaaaaaataaatccattcttacttgaatgtatatgcacattaaactagtattaatctaggaaaaataataggtagaaacatcattttggtcatgaaagtcatactctaacaagctcaactcaaacttaaacacatgatgacttgcaattgccttccttcctttggcacatctaaaccacacagaaatcatacattgcttggttaattcttgagggacatatttgcatcagaatttaaagatggattttaatttttataacattatattaagacttttaaaaactcaatattttactcaataggtttgcagcaagaaaggttgtgttcttgaaatcgtctttggagcatgtagaactcatgatcttgaaaaataattcttgcatcaaagaaaatctcaattctctctgaagtctttctaaaatacaaatattttattccaatgttttgacattctaatggctcagaagaacaatttatatgtccttgtagctgtgctcctctttgagatgtgacctgcaacagggctcaattgctttactattagttctccatttccatgcttcatttccttcatgtagctcgggctggagaaaaatcagcatgttctgatgagtttaatactatgaggcagtatgatggacctgaatttagtggagattggagctccaaaataaatacaacaccatgtgtcaaataaaaaagaaaagatattctcctgtacaaatcagaagagataataaaaatcaatgaacagacagcaacttttttttttatcatacctacacaagcatctcaaaactatcaaattatttacctttttcttatttggaacacttcataatttattggataaacaatggtttatattgccttaaactaaattttactggcttttgtggtagggttttcagttaggaaggaatttctgggaatttatatattcctaaataaaatatttctgttaatcaagagcaacataattctgttggattctataatatagtaagctataagcatctctgtaaattaaatttgtcccaagttttgatatgcaacaagttccagggtttttcaatagctcatcatgttctattcctctcaatgacagtaccatgaaggtatgtacagggcatctttgactcactgacaacacagggcactactttctcatagaggtttggtgcctttgcaggtatatgagagttgctatctattcacaaaccactgagcatttatttttatcaaaaaaccttcaaatgctcagagtctgtggtcagtgcagtcctttagataagtctaatgaagatatgcctcaccaaggcagaaatctaaacaattaaaaatggagaaatatttacaaccatctgtctccagcaaggggagttcttgttttctgtatgtagtggtttattattttatttcattttattttattttttgctgttactttttcttcagtacatttcgaattaaggttccaaggctatgagtacaaactctcttggccagtcccatacatgtccgcgagtcgtttaaagcgaggtccccagtcacttaggtagtcatagttctgatcagagtttgagctgatggaatctaaagagctgagtgattcagcaactgagccatttccttcaaaagcatatgtctgcagggagtcataaggaggagcaccaggatcaacatcggcttcttttaatctttcccaaataaattccctaaagatgacattatctgggatgcttttaaaagctggtcgactcaggaattgaatttctggagtcacatccctccgggtcttggtgtctcggatgacgttgaggtttctcagtgcagccatgtcaaacgcttccgtgtcctcctctcccccgccctcgtcatcgtatctcacaatattttctctgatgtctctttcttcgtcaaaaataaggggctcttttttccgtcttctcatagtgacgataaggaggatcaacaccaataatgtcaagacacaggcgagtatggctatcagggctcctgtactgaggccagcaggtaggacataggcctctgcattgcaggtctgggctacgccgtcagcatcacagtcacacacgcggatggtgagggtgttggtgctgctaagtgagggagatccactgtccacaatgaaaattggcagatagtaaactgattgttcctgtctccggaagccgtttctcctggtcagtattgaggctgtgttgtctttgttatctttcaatgaaaagttgtggttatttgttgcatccgttgttaagctgaagtaaaactggtgtccattggatggctcatctttatccacagcactgattttctggataacctgccccggctgggcattttcacagacggtggtctcatagtccatggcaaattcaggggcgttatcattgatgtcaagtatagtgatggccacatagcctcttcctacttgagatggattctggctctccattgcaaggactgtgatattgtgaatagcatttgtctctcgatccaaagacttggcagttgtgatgaccccactgttggcatcaatattgaagtatctctccaagtctgtgtttctgtcaattgagtacctcacagggctattggaagaatctgggtcatgagctgctacagtgccaatgatattcccaacctgggtagcttccgacacctccatagggtacaagggtgaagagaacacagggggctcatctacatcttccacaattatcttcacagttgtcgtgtcactgaacggacccaagctcagaaagcgagggtcggcatctttatttgcagcttctatccgtagcgtgtaacttgttttggcttcaaaatccagctccttctgtatagtaatgattccttcctgggtttctttgtcaacagaaatcttaaaaatgcccaaaccatcaccatccacaatcttgtactccatttcagcattagctccaatatctgcatcagcagctttaattctggccacaactgaggctacaggtaatgactctgggacgttatattgataagaccttcgaggaaagcgaggtggattatcgttgacatcagttagggtcacagtgactgatgtagttcctgacagtcctccattttgaccaaccatatcctttgcctgaatgacaagcaaatactggtctttagcctctctatccatgtttggaagggcagtcttgatgactcctgtctttggctccactgagaagtacggctgtccttgcagaatactgtagaccactctggcactgttgccatatgtaggatcatcagcatccgtcgctgtcacttgtaccactgaggtccccacgggagacatttcgggaactcctgccgtgtatgggccatccaaaaatttgggttcattgtcgttgatatcctgaattttgatgacaaactccgactcgggctccacgggtttgttggtgagcctatccagcgcttgagctcggagcgtgtagtaggcctgctcctcacgatccagtctcttggtggcatgaatatccccagtgttctcatcaataatgaaaatggaacttgccccttcgcctgacaagatgtatttgatggaaccatctcctttatcaacatcagagtgaagctttcctacatagagggggtctgaacccatgtattcctccagcacaaagaactgattccacacccagctgcgcttggtccgggacctccctgattggaaatagggctttgatctggaccttgagagttctgcttgactcatcccagaaaaacacaggaaaagagctattagctgcagaaaatggcagaactccactttgcccaacttcatcttttttttttctttctttttcctgtgtaagaaaaaaaccttgacaagagaaaaggcacagttccagttggcttagtagctcttgcctccggcagggtgtcagctgggagtccagagataataatctgtagagtgttggattggaagaggtcaccactgctgaatagccttcgccaaagaatggtgtagtaagtacctggggcctcgctgccctccccacggcgtcagacgccagggacccgggcgtgtgcatccgaaagaacgtgcgctcggctgccggacgcccgcgggctcttggggacccagtgcgcgcagctccgcgcgcggggcagact

SEQ ID NO: 18747 - RNA, 10570 nt, Homo sapiens
  source 1..10570: mol_type = other RNA
tgagtgtgtgtgtgtgagtgtgtgtgtgtgtgtgtgtgtttgcataagttacagttattctgggcatcaaagtttttccttaaaaaacctaacaatgcctaacttgagtgattcacagacttataagaaaattgaaaccatgtatatgttagaatgttatctaacttaaaattacatatctgtggaaaaactttattgtgatacttttatattaaaaatcagtcacttagaagaaaatatcaaactttaattacaatgatactcattttctgtaccgagttgtcaggaggtataagctggaaaccaggatggcgccaccatcacagctgagaatgatgacaacagaagtcttcattgtagtgtgtcaggtcttttgaggtaccaagaattgcggaaattattttcttctatgtatcttactctgtgataattttttcttattttttaaaaatacagcaaaacacacaataaaacacagcaatatactgaggtctcacattctcacggcttgtcttcctacacttattccaattcagagtacactttgtatacatctcttcgctggttagttctgaaacagtactctttcttatatttgttttaaacatctccaatactgaatattgtaggagtctatttgcctgaaagatagcacttgagctgaacgaaaataatctattcagtttggacatacatcctgaccccaggttttatgcttcatgtctcatttccaaggttaaatgaactggattttcaggatcaattctgcagtcaattgaattaacatttttaaggctcttttactatagaagtgactcttacataagcaaaaatattataaaagtggttttctttttaatgtaattataatggaatctcataaacataaaaattatagtttcattgaaagtaatgctgtgtgttttactaatgtgaattgttcgttcctctaaatttgagaaaaaaaattctgaaatctctactaaagagaaactttacaaatgtgcaattctccctcagtatgctcatataatttaattgtagaggttggatctaatagacatcttaaaagctaaaaagaaaatatttaaaagtcatttactttacttcaacatttcgcctcaaattgtgtgtgttcctgcacacgtgtatgtatgtgtgcgcatgctgtctatatatacacacacacatacgcacacaaaattcaaagacaaatacataatatatataagttgtgtagtgacttatttttccttttccttttatttttgggcatttaaaattactgcatgtaaaatgaaattgctatatagttacacaggaaggggaacaccacactctagggactgttgtggggtagggggaggggggagggatagaattaggagatatacctaatgctaaatgacgagttaatgggtgccgcacaccagcatggcacatgtatacatatgtaactaacctgcacattgtgcacatgtaccctaaaacttaaagtataataataataataaaaaaacttgattgttcttaaagtattggtcatatacagtatacaacatattccagatcttgatatacaaaaacatagggtttatactcacaaaattagaacatgaagctgtagggtagtgaatcatataagtttttcctgcttatataaaccattaacatcattatattcattaataaaatgaaaatgcaagtttgtttttgaatgaaagtatgctgtactttcaacattctcattagttacatagttattaatatatttgtttctagtgtctgttcacatgagcataaaataaccagataactaagagctaaagttgagaagagagcttattaacattcatcttggcatcactgacaaaaagtaatatccattatatattattttttagtttcctagagtttcttcattcgtaagagattaagatgagctgttgtaagatataagtgagtttgagtcatcaagagtgcattgcattcaggatggttttcatgttaagtcaatatcattgcatctaattttttcaagtgtataaattattaattacacatatgtcactgtgactttaaaaagtattgtattctctagaacttcattttctttatctactctggatgcctggaagaccacttaacttatactcattattgtctttttctctattctggtgttttgtgttcatcaatgaggctgggatcatctaaaggcagtcctttatcttccactcagttatcattataagtaagaaagatttgttctttatttataatcccattcacatatggatatcattaattcatatgaatggttgaattatgttgagttaaactgcaatcttctgagatcttataaataactgtatttgagtggcttcaattaattatgacaattatctatttgaatattattttccaatttaggataccaagttgcatatatttttccttaatgtatgtatctccaaacagaaattctctgtttaccatataacaattatcaacctttttatataattcccattatttcccataataaagctttatctttttatagtgttttactgtttacacagtctttcacttaatcattcacaagcctctgaaacacaatagtaattaactcaattttaatcatgaagctataaaagttcagagaatgaaaatggcatctagggcacagcaaaaatgtggcgaaactgagcttctgacctagattttataaccacagaccagaggtaatttctggtataccacactgacaccaaagcccagtaacatttaataacaaataattcacactctatattctgttaacaatgagattaaatctgcacaataatatgtgacaattacacaaataacagctaaatgttctttccttagccaccaaaatccttaccttaatataaattagattgttacagcaaataagatatttctcctttcattcggtaccatattttctagtcttattgcctaacagtcacttggcaggtgacaacaatacgccagcattaaccaggaattatgagactcttatttttacattacttcagatacatctctcaaggttcccaatcacacacatgaaaacgcacacacagggccgggcgcggtggctcacgcctgtaatcccagcactttgggaggccgaggcgggcgaatcacgaggtcaggagatcgagaccacggtgaaaccccgtctgtactaaaaatacaaaaaaattagcggggcgcggtggcgggcgcctgtagtcccagctactccggaggttgaggcaggagaacggtgtgaaccctggaggcggagcttgcagtgagccgagatcgcaccactgcactccagcctgggcgacagagcgagactccacgtcaaaaaaaaaaaaaaaaaaaaaaacacaggcacacatccttttcagttacattctaagccagtagaagttagcataacaatgaaaaagtgtcagaatgcaacgcacactgcctgtcttgatttgcttgaaaaatttcccacagaattatacgttacaatgtcggccaaatcacagccttaaacatctcccatttttcttaagggcttatcccactcttctgaaatagtttcaattacatttaaaatgcaaatgctattattcctttcttgttctttattatatccagccgactaacatgattgtattagctttcattgccaactttcatacaccgtcatatatacacacaatatacattattaataattaaaaaataaacatacactaacagaaaataaattggtttatctattatttgtcatatatatttcacttgcctccaggcatcgtggaccagaaagagttaaaaaataagttgaagctttcatcaacttcaattggattaggtcaactgtaaataaaactttaaatggtgacttggaaaataattagtgttattattagaacagtttgtaagtgaatacatgttaaattgaaaatctgaagattaatatttacagctagtgctttaaaactttaacatgtttaaatcatttagcttcttgcagtttgtttagcttagcttattttaagctgctttagattttatatttcaatataaatgctaacaacactatttgcatttgcatttcttgggcatgtggatcacttcacaaatatcattcctacattgtgtaactatgccgttgacatgaaaataattgcctatgtctaccatccaatgtagtaaatgtaattgtgcatgaagataaaataatttaaaacttcctcagagggcagagtgaaaaggcagctaccattacttaaccactactacctcctgcatgtatcttgtagacaactaacctcaattgtagtcatcagcagagcttcctggcaaataaagacatttaccagatcccagatctggtgattgcttgtagaaaaatcaaaaatctacttattgcctgcaaattactacctaattttttattgatgtctctttcctgattttgttccttagctggctgatcttggaatatttctttcagagactaatttgtgaattgagattgataatttaggcttgatctccagaaatccatttccttaagatttgatttttatatttttatgttgatttttaataatgcaatggtgacaattcagattaagggcttgggtgtatttccttgacatagacagtaagaagtaaaatgcatctgatttttcaataaattaaactgttcaaaatgggcataatttggcaaaccctgagtttctattgatgctcctgtatggacaagtggaaaataattaaatatattgacttcctgaactattatctctacttgaaatttagccattgttttccataaagaagtgactcctctccctgtctacaagtagctccaaggatttcacttcaggaaatcactaccacatacattgttatttagtagtaaaatatagcataaattcctttcatgtcattattttaaatcatataaattcatactatatttacaattatgacatttcattttataaaataatttaagcagtagagtgctggtaaatgtttaacaacttgttctccagagaaaagggtagtgtttgctgattactgttgtggtctaaataatcccaccaaggctgacatcaacctaccaaaatgatatcactgtacctggagttgggaagagatatgaagaattagttcctgtgagctcattctagttggtttcagtataatactgaatttaagcaacttgataatatatatttatttaaatcatatttggagaattttccaactagacttaatattaattttatcaatcagctcttcaatcactgtttttaaaacaaagcctatatctcaagtattgacagtcatcatatatagcattagatttcagaagaaaaaagaaaactaaaataagcaacggcaaaaaatttactactattacaattaagcttagaatacttcatataaatactacctatattaggaacattcttccagccatctcaaaaattaattttttaaattaatttttttaattaaaaaataccactgaatgaaatgtaatactgtattcatataatcatccacacataaatagcaattgggtatatgcaataattttaaattattatttaaacatgaacctttctttttccaatctatcattggtaaccatttgaaaaaattaatgagaaaaaacacacattttaaaagcagaaaaagcagggtgaatgatgtgtgttccttttctaaaatacatccacacctccgtttagtggtatgtgcaacaatcagcagttttgacatcatccaaatgtactaaactatttcatcttcttgcagacaacaaggggattattacaaactgttttctcagcaccttgctgacttaacaactctgtaattcctgcaccacactctgattttattgaactgggtaaatacgcgtgtttttttgtttgtttgttattttttagtttgaaaaacttgcatgtgtgattaaaagttatgaacagtatctttcactgttataattttttaaaatatatatgcatattaatacagcaagaagcatatctatatagtcataaaacaatgtctacaaaactctattcaaattaaagaactgtttgcaggtaatgaaatttattggattatttatacttatgaagttgaaggccacttttacatacttcatttctaaagttgggctgcaagtttacagaatcctacatagttcttctttgtgtaatcaacatattaatattctaattccactgtctacctttcaaaaagcacttttagaacatgattctctacacagtgtttactatctgtaaatgtattaggaacccaacaatgaattatttttaaaaggagaaaggaaggaaaaaataaatccattcttacttgaatgtatatgcacattaaactagtattaatctaggaaaaataataggtagaaacatcattttggtcatgaaagtcatactctaacaagctcaactcaaacttaaacacatgatgacttgcaattgccttccttcctttggcacatctaaaccacacagaaatcatacattgcttggttaattcttgagggacatatttgcatcagaatttaaagatggattttaatttttataacattatattaagacttttaaaaactcaatattttactcaataggtttgcagcaagaaaggttgtgttcttgaaatcgtctttggagcatgtagaactcatgatcttgaaaaataattcttgcatcaaagaaaatctcaattctctctgaagtctttctaaaatacaaatattttattccaatgttttgacattctaatggctcagaagaacaatttatatgtccttgtagctgtgctcctctttgagatgtgacctgcaacagggctcaattgctttactattagttctccatttccatgcttcatttccttcatgtagctcgggctggagaaaaatcagcatgttctgatgagtttaatactatgaggcagtatgatggacctgaatttagtggagattggagctccaaaataaatacaacaccatgtgtcaaataaaaaagaaaagatattctcctgtacaaatcagaagagataataaaaatcaatgaacagacagcaacttttttttttatcatacctacacaagcatctcaaaactatcaaattatttacctttttcttatttggaacacttcataatttattggataaacaatggtttatattgccttaaactaaattttactggcttttgtggtagggttttcagttaggaaggaatttctgggaatttatatattcctaaataaaatatttctgttaatcaagagcaacataattctgttggattctataatatagtaagctataagcatctctgtaaattaaatttgtcccaagttttgatatgcaacaagttccagggtttttcaatagctcatcatgttctattcctctcaatgacagtaccatgaaggtatgtacagggcatctttgactcactgacaacacagggcactactttctcatagaggtttggtgcctttgcaggtatatgagagttgctatctattcacaaaccactgagcatttatttttatcaaaaaaccttcaaatgctcagagtctgtggtcagtgcagtcctttagataagtctaatgaagatatgcctcaccaaggcagaaatctaaacaattaaaaatggagaaatatttacaaccatctgtctccagcaaggggagttcttgttttctgtatgtagtggtttattattttatttcattttattttattttttgctgttactttttcttcagtacatttcgaattaaggttccaaggctatgagtacaaactctcttggccagtcccatacatgtccgcgagtcgtttaaagcgaggtccccagtcacttaggtagtcatagttctgatcagagtttgagctgatggaatctaaagagctgagtgattcagcaactgagccatttccttcaaaagcatatgtctgcagggagtcataaggaggagcaccaggatcaacatcggcttcttttaatctttcccaaataaattccctaaagatgacattatctgggatgcttttaaaagctggtcgactcaggaattgaatttctggagtcacatccctccgggtcttggtgtctcggatgacgttgaggtttctcagtgcagccatgtcaaacgcttccgtgtcctcctctcccccgccctcgtcatcgtatctcacaatattttctctgatgtctctttcttcgtcaaaaataaggggctcttttttccgtcttctcatagtgacgataaggaggatcaacaccaataatgtcaagacacaggcgagtatggctatcagggctcctgtactgaggccagcaggtaggacataggcctctgcattgcaggtctgggctacgccgtcagcatcacagtcacacacgcggatggtgagggtgttggtgctgctaagtgagggagatccactgtccacaatgaaaattggcagatagtaaactgattgttcctgtctccggaagccgtttctcctggtcagtattgaggctgtgttgtctttgttatctttcaatgaaaagttgtggttatttgttgcatccgttgttaagctgaagtaaaactggtgtccattggatggctcatctttatccacagcactgattttctggataacctgccccggctgggcattttcacagacggtggtctcatagtccatggcaaattcaggggcgttatcattgatgtcaagtatagtgatggccacatagcctcttcctacttgagatggattctggctctccattgcaaggactgtgatattgtgaatagcatttgtctctcgatccaaagacttggcagttgtgatgaccccactgttggcatcaatattgaagtatctctccaagtctgtgtttctgtcaattgagtacctcacagggctattggaagaatctgggtcatgagctgctacagtgccaatgatattcccaacctgggtagcttccgacacctccatagggtacaagggtgaagagaacacagggggctcatctacatcttccacaattatcttcacagttgtcgtgtcactgaacggacccaagctcagaaagcgagggtcggcatctttatttgcagcttctatccgtagcgtgtaacttgttttggcttcaaaatccagctccttctgtatagtaatgattccttcctgggtttctttgtcaacagaaatcttaaaaatgcccaaaccatcaccatccacaatcttgtactccatttcagcattagctccaatatctgcatcagcagctttaattctggccacaactgaggctacaggtaatgactctgggacgttatattgataagaccttcgaggaaagcgaggtggattatcgttgacatcagttagggtcacagtgactgatgtagttcctgacagtcctccattttgaccaaccatatcctttgcctgaatgacaagcaaatactggtctttagcctctctatccatgtttggaagggcagtcttgatgactcctgtctttggctccactgagaagtacggctgtccttgcagaatactgtagaccactctggcactgttgccatatgtaggatcatcagcatccgtcgctgtcacttgtaccactgaggtccccacgggagacatttcgggaactcctgccgtgtatgggccatccaaaaatttgggttcattgtcgttgatatcctgaattttgatgacaaactccgactcgggctccacgggtttgttggtgagcctatccagcgcttgagctcggagcgtgtagtaggcctgctcctcacgatccagtctcttggtggcatgaatatccccagtgttctcatcaataatgaaaatggaacttgccccttcgcctgacaagatgtatttgatggaaccatctcctttatcaacatcagagtgaagctttcctacatagagggggtctgaacccatgtattcctccagcacaaagaactgattccacacccagctgcgcttggtccgggacctccctgattggaaatagggctttgatctggaccttgagagttctgcttgactcatcccagaaaaacacaggaaaagagctattagctgcagaaaatggcagaactccactttgcccaacttcatcttttttttttctttctttttcctgtgtaagaaaaaaaccttgacaagagaaaaggcacagttccagttggcttagtagctcttgcctccggcagggtgtcagctgggagtccagagataataatctgtagagtgttggattggaagaggtcaccactgctgaatagccttcgccaaagaatggtgtagtaagtaccttagcctgtcgtgaaagccgtgatcagttgagctcctgaggcatgaaggcaaagtcataaaactaatcagaacttacagttttcttgcttgatagttttgccctttcaatctcctcggactgccctag

SEQ ID NO: 18748 - RNA, 507 nt, Homo sapiens
  source 1..507: mol_type = other RNA
tgagtgtgtgtgtgtgagtgtgtgtgtttcaagggagatttctgagctgacagtggtgtcaatgtgtgagtgtgtgtgcatgtgagtgtgtgtgagtgtgagtgagtgagagcatgtgtgtgtgtgagagtgtgtgtgagagtgtgtgtttcaagggagattcctgggctcgggctcttggacattgggcagaaggctgtgtcctctcctttgaccagtctctgttgtgtttcttccctgagctcatcaagagcagcctcagccatcccaagagcccccagagctgtttgtgggcagctgagcctgtgcagcccagcctcacccttgtcacagtgggccctaccaccatgtttggcccccatgagccatggcattttcacagtcaccctgcatagaaccaaggctggtcaccctttcacagatggagacacaaggaggatgtagcagtagggtgagatcagatcacgaggcggcttttgcttgttttttgataagaaagttttattt

SEQ ID NO: 18749 - RNA, 853 nt, Homo sapiens
  source 1..853: mol_type = other RNA
tgagtgtgtgtgtgtgagtgtgtgtgtttcaagggagatttctggatgatggtggtgtgaatgtgagtgtgtgtgagtgtgtgtgtgtgagtgtgtgaaagtgtgtgtttcaaaggagacttctgggatgatggcgtaaatgtgtatgtgagtgtgtatgtgtttcaagggagatttctgggatggtgtcatgaatgtgtgcgtgtgtgtgtgtgtgtgtgtgagggttcgtgagtgtgtgtgtttcaaggaagatttctgggatggtgttgggaatgtgtgtgagtgtgtgtgtgtgtgagtgtgtatgtgtttcaagggagatttctgggatgatggtggtgtgaatgtgtatgtgtgtgagtgtgtgtgtttcaagggagatttctgagctgacagtggtgtcaatgtgtgagtgtgtgtgcatgtgagtgtgtgtgagtgtgagtgagtgagagcatgtgtgtgtgtgagagtgtgtgtgagagtgtgtgtttcaagggagattcctgggctcgggctcttggacattgggcagaaggctgtgtcctctcctttgaccagtctctgttgtgtttcttccctgagctcatcaagagcagcctcagccatcccaagagcccccagagctgtttgtgggcagctgagcctgtgcagcccagcctcacccttgtcacagtgggccctaccaccatgtttggcccccatgagccatggcattttcacagtcaccctgcatagaaccaaggctggtcaccctttcacagatggagacacaaggaggatgtagcagtagggtgagatcagatcacgaggcggcttttgcttgttttttgataagaaagttttattt

SEQ ID NO: 18750 - RNA, 3582 nt, Homo sapiens
  source 1..3582: mol_type = other RNA
tgagtgtgtgtgtgtgagtgtgtgtttgtgtgtgttcatttggaaagctaaacatgaaactattaacagtagttacttttaaagataagattactgtgcggatggtgcggaagggtggtgatgttctgtactgtttgtacatttacaacatgatgtattacatggataatagaatttttaagtagcaaggagatttccagtttgaaatataaaaggggagaaaaattccaaatgaaatggaatctcccaaattgataaagaaaccgtgtgatcctggagggtgaacagggacctgggaatcaggcctttggccattgtctatgatgctggacccagtggctccattccaccctagtggcaaggccaagaccgaaatctctccttgaggcttgaagtaaagagccagctgaagaaatgccagaggcaccagatctttggagataaacagcaggctcagttttgctgcaggggttaaatgtagccaaagaagtgatggtggaaggtgtggtagctccctcagggtaaacagatacagtctttctattcattcaaactaacagactcagagaaatctcgcagtggaagaaccttaatataacctagtgcttttggtcaagaacagacccagaggaactcatcaacttattcaaggtcaagcgtgtcgtgaatgagagaagggatgagatgagaaccacatcccaggtcttccccaacggtcttcttgaccctggaagaagactcactctttgtgtccctgaagtttgtctgatgatgcaataaatcagaaaaaggcatctttttcctgtgtctattgacgccgtcagccagcatgactcaaaaggtagggagtgttaagttgggcagttcgtcacaaattttgatgacattttagatacgtagctggagaaaatacccagcactcttttcttctgtgttttctcatctagtaaaccttcttcctgacatcctaggagcacctctgtttagagaaagagaaaacgagtccttggtgtactttttttgtacacttagcataacttaaaatatcaatcacttccttcttagtagagaagacggactacaatgatggcatcaggagtgctggaattggttattgctggaaaacatagaatgggaagcccacatctctcatgtgtgacccacttattttatgcccccgctttcttcctctgatctttcaatactctcaaggcatcttatccaattcctccattctttctcatttcccattctgtgtaccacgtttggtcctaaccccctccacttgcaattctctcccagttctccctattcctcatctttccacttcattttcctaccaactctcctcctccagtcttgttttgcttccctcttttgtgtcttttctctttatctctatcttactgcatctattcaatccctcacccccataaaatattatagagaagccaagtcacaggtgccagtcaaaggaaagttttaggaaaatgcatttggaaacagcagtggcacagcagagttgccaggaatgggcaatgagtcctaaatgggaagctgaaaagatacagcgaaatcatggctggtttaacttcaagcaagttgagctaatgctctgggtcagagccacactcccctactgagaagggacattcagggtgactcctcaccatatgacttgcatttatagttatggattatctcagcaaggaggtttggagactaagagtgagagttttggagaaattttcatattgagtagtcttggattttctgaaatatgtaaataatgcttagattataaattcttatcttttcaaaaaatttgaaacacatgggagaaaaagatgaggaaaattcatttttgtaacataagatatataatacatattaatggagttttagcatttggaaacaagtctgtgagctgcacacaggtatcaggtgctccagaattactagagaatacataatcatacagcttcccctctgtcccctgtctatgctatggggtccttgtttaatgggaatagaaagagctacttttttgtttttgtttctttttgttttatttttgcttttagagttctgatgggagaaataaaacaatcctaatctctagacctatgttttataaacagaccaagcacacctgaacttgagggaaaaatatgacttctggcggggagttttctggggtacttctggcaactaaggctgtaaccaaccaaagagtcattccttctggaacatgaacctgtcagcactcacagcttcctaggtttcacctctagccagaaaggagagaacacggtgcctgaagctgaatttgtctaaggggctggcttggcagatcctatacactcattgcttataattggacagggctgctttcagaaatgaaaactattattccctacaaaaagtccttcttatgcccatgaaacagaaacaggtgtgaaccatttttttcctagtttctggctctagaagacttttcctttagtacaagacacagggagaaagggtcaattgagacctcctcaagccagtgaccgcctccctgtgagcatcctccagatggcactctgcacatcagggtttctgaagctgtagatgattgggttcagcatgggattgatgacagtgttgaaaattccaacagctttatccttgtctgaaagcttggttgaacccagtcgcatatagttaaagatacctgaaccatagaatatggcaaccacagtgaggtgggagccacatgtggagaaggctttcttcctgccctctacagagcgaattcgcaggactgcagctgccacgtggatataggagatgacaatgagagccatgggggtacctgccattataaaacccacagcaaaaagcagcagctcattgagttgggtgctggagcaggagagctggaagagctgtgggaggtcacagtagaagtgattgatcacattggggccacagaagttgagcgtggacatggccacagtgtgggtcagtgcgttggtgaaagcacaagcccaggacgcagccaccaacatcctctggactgtctgactcatgcgggtgctgtaggtgaggggccggcagatggccaggaatcggtcataggccatggcggtcagcaggaagcagtccactccaacgaacagatggaagaagaagagctgggtaaggcaggccccacagggaactgcacgcttgcgggacaggagacgactcaacattgatggaacagtgacgctgatgcacccaacatccagcactgataggttccccaggaagaagtacatgggggtgtggagtttgggctccaccaagacagctgccaggatgctgaggttgcccctgaccgtgaccaggtaggcaaagaggaagagcacaaagacaactggctgcagccctggcgcctccagcaagcccagcaggatgaactcagcaatgactgttccattggccccagattctggctgcatgagttccacaccaatgaagtccagagaatttattcatcttcacaaagccacagtggatctaatggtggtgctgaggctagagtaagtatcc

SEQ ID NO: 18751 - RNA, 2899 nt, Homo sapiens
  source 1..2899: mol_type = other RNA
tgagtgtgtgtgtgtgagtgtgtttaaaaaatctgtcccaccacacaaacttctctctataaagcagataacagggaagaacaataacaaaagcaaaacaagccaattgctctctctttgggatatgattatttcccttgtgaatgaagtattcaacaacataagaaaaggaaaagaacgatttcttttgtatactccctaaacacacagagtttactgggtcagatttaactgtgagcatttatatgcctacttccaggcatcgtcatctgatgtttcactgctactggtttcggtgtctgagtcctcaaactctgctttgcaagtgcttctccaaggggagaacagactggaactgcggctctgcaagaagccattctttccaaagccatttcttctcagctgctctgtcttcatgtggaactctttgagctcatcctctgtgaggggaaggcaattctcatcattttcaggatattcctgccaacccatagctttcaataacctgtgctctgcttctagagagtgtgagagaacctccccttcttccactacagggagggcaagaccattttgatgacagccttcctccccattttcctttggttcaggtgtgctgttgtcctccaaatcttccagcttgtcacagtctctattctctgagaagtctccattccggtcatccttcagagttttcaggaactcactcttcctgtcggtggttcggcgggtcaacttggtcagacgagaggagctgatctcaattggaggggtggtgctggagggactctctttgggagaactcagagctgcaccactagccagtaccactggtttggtaacagagattggactggtaaaagcagactcccggctagaggaaagggatcctgacttgtgctccatcctgttagctttccatgcattaggcttggaaggaggtggtacaggcttaggaaccaggttcttatagacacttggaaccacggatgacaatttgttcccatttgcatggtgagatcctggtgaggtgaatgcagcagagaaggcagcagcaggatcctctttggaaacttttttgataactagcatcttggagggttgcttggcactaggcgggttttcccatactccagaaggtgtcccaataggtctgcatggctgatgctgtttgccagcttctggattcaaggaaggaaagtcctcctcttcaaactgcaacttttccaccttgtcttctttcttttcttccctaatctccataggtggcttttcctgaaaagcacaccctttccgggagtggaagctgccattccaatggcgatggttccctgtgccacctccactacgttggctcatgccatcatgacctcgggaagagctatgccaaccagatgggttccctgtgattccagcatatgctcccttagagacaccagagtccacagaatcatggcggaacagggagggctggtgccaagaatctcctgcagttcgtaggggaccattgttaaaaaaaccatcagaggaattatgtcgacggcggcttactccaaatctaccttctcctctgggtaggtgctctccgtgtttttcgaaggtggcagtaggtgacttagctgactgtggtgttgagaaatttagccaagcaggaacaaaatcatgctgcgccatttaggtccagtgtctcctttcagtaaggtgaggcatccaacctcatggccaggatcccagagtgtaacctctgtggtcctgtttctgaactcgagtcggccagctggatctcccacaaggtttccttgttaaaagggtgcttaagtaacctggccggcagcacgacttatgatgaagcacgaagaagccaggttctgtgtcgatcactctctcagtcccctcaactgctcatcttaaactatttggttcctgacacgtttccaaaaggggaaaggggaaaaggggaaggggggaaggggaacataaaaagtatttgttacatttaaaaagggggggaaggggaaagagctgtatctatgttcacctcattcaacttccttgagttatggcactatgatgttgcttaattaggtaagacatggatatttgcaccgagtgcaaatactgttcataacaaggtcatagctagaaagacagatgggctcaagtgtggacaaataatgtcatcaaggtaatagatcaaaaatattaaagccctataaaagatctgagcagtcaactccaaaacatccacatgacaaagtccttaaaatacaaatctcattactcttactcatgcaactgctaaaaaatagtgtgcagatatgtatttatatttgccttaaccttcaaaatctagggacataaatcttgtctttgttaaaaaaaaataaaaaataaaaatagacaggaatttgctacacttttccctccacgaacagcagctttcaaggcaaatttcttggtataaagctactaaatgtatattctatgtctttggcctttactatttataaattcagagcaaagttaaaacattagaacgatgggtaggatggatattaagaaatagtcaaggagaaatataggtccaaaatgaggatttcttctcttcagttttctgtgtttcacttgttctgctccttcccaaaatctaaattgagccactggaaggagatatgaagaatcttctatgctttggtagagaagtcacttattattttggatccatttccaccacttcacaatcatttgaaaggccacacgaatctatcactccgaactctgtgggcagattctgctgcctgggagccctggaatagaacttcaaggaccgttcaacatctggattcaactagaaattaagaatggcccccaaacagaaagccgggcctaggaaccaatt

SEQ ID NO: 18752 - RNA, 2902 nt, Homo sapiens
  source 1..2902: mol_type = other RNA
tgagtgtgtgtgtgtgagtgtgtttaaaaaatctgtcccaccacacaaacttctctctataaagcagataacagggaagaacaataacaaaagcaaaacaagccaattgctctctctttgggatatgattatttcccttgtgaatgaagtattcaacaacataagaaaaggaaaagaacgatttcttttgtatactccctaaacacacagagtttactgggtcagatttaactgtgagcatttatatgcctacttccaggcatcgtcatctgatgtttcactgctactggtttcggtgtctgagtcctcaaactctgctttgcaagtgcttctccaaggggagaacagactggaactgcggctctgcaagaagccattctttccaaagccatttcttctcagctgctctgtcttcatgtggaactctttgagctcatcctctgtgaggggaaggcaattctcatcattttcaggatattcctgccaacccatagctttcaataacctgtgctctgcttctagagagtgtgagagaacctccccttcttccactacagggagggcaagaccattttgatgacagccttcctccccattttcctttggttcaggtgtgctgttgtcctccaaatcttccagcttgtcacagtctctattctctgagaagtctccattccggtcatccttcagagttttcaggaactcactcttcctgtcggtggttcggcgggtcaacttggtcagacgagaggagctgatctcaattggaggggtggtgctggagggactctctttgggagaactcagagctgcaccactagccagtaccactggtttggtaacagagattggactggtaaaagcagactcccggctagaggaaagggatcctgacttgtgctccatcctgttagctttccatgcattaggcttggaaggaggtggtacaggcttaggaaccaggttcttatagacacttggaaccacggatgacaatttgttcccatttgcatggtgagatcctggtgaggtgaatgcagcagagaaggcagcagcaggatcctctttggaaacttttttgataactagcatcttggagggttgcttggcactaggcgggttttcccatactccagaaggtgtcccaataggtctgcatggctgatgctgtttgccagcttctggattcaaggaaggaaagtcctcctcttcaaactgcaacttttccaccttgtcttctttcttttcttccctaatctccataggtggcttttcctgaaaagcacaccctttccgggagtggaagctgccattccaatggcgatggttccctgtgccacctccactacgttggctcatgccatcatgacctcgggaagagctatgccaaccagatgggttccctgtgattccagcatatgctcccttagagacaccagagtccacagaatcatggcggaacagggagggctggtgccaagaatctcctgcagttcgtaggggaccattgttaaaaaaaccatcagaggaattatgtcgacggcggcttactccaaatctaccttctcctctgggtaggtgctctccgtgtttttcgaaggtggcagtaggtgacttagctgactgtggtgttgagaaatttagccaagcaggaacaaaatcatgctgcgccatttaggtccagtgtctcctttcagtaaggtgaggcatccaacctcatggccaggatcccagagtgtaacctctgtggtcctgtttctgaactcgagtcggccagctggatctcccacaaggtttccttgttaaaagggtgcttaagtaacctggccggcagcacgacttatgatgaagcacgaagaagccaggttctgtgtcgatcactctctcagtcccctcaactgctcatcttaaactatttggttcctgacacgtttccaaaaggggaaaggggaaaaggggaaggggggaaggggaacataaaaagtatttgttacatttaaaaagggggggaaggggaaagagctgtatctatgttcacctcattcaacttccttgagttatggcactatgatgttgcttaattaggtaagacatggatatttgcaccgagtgcaaatactgttcataacaaggtcatagctagaaagacagatgggctcaagtgtggacaaataatgtcatcaaggtaatagatcaaaaatattaaagccctataaaagatctgagcagtcaactccaaaacatccacatgacaaagtccttaaaatacaaatctcattactcttactcatgcaactgctaaaaaatagtgtgcagatatgtatttatatttgccttaaccttcaaaatctagggacataaatcttgtctttgttaaaaaaaaataaaaaataaaaatagacaggaatttgctacacttttccctccacgaacagcagctttcaaggcaaatttcttggtataaagctactaaatgtatattctatgtctttggcctttactatttataaattcagagcaaagttaaaacattagaacgatgggtaggatggatattaagaaatagtcaaggagaaatataggtccaaaatgaggatttcttctcttcagttttctgtgtttcacttgttctgctccttcccaaaatctaaattgagccactggaaggagatatgaagaatcttctatgctttggtagagaagtcacttattattttggatccatttccaccacttcacaatcatttgaaaggccacacgaatctatcactcgggcagcggcggagctatggccagggactagacgctgcgtctgaggacgcgtccccagcttgtcgacccggcagaggcggctagtccacaaccataacaaagctcttcccaaaatggctgcccggcccac

SEQ ID NO: 18753 - RNA, 2881 nt, Homo sapiens
  source 1..2881: mol_type = other RNA
tgagtgtgtgtgtgtgagtgtgtttaaaaaatctgtcccaccacacaaacttctctctataaagcagataacagggaagaacaataacaaaagcaaaacaagccaattgctctctctttgggatatgattatttcccttgtgaatgaagtattcaacaacataagaaaaggaaaagaacgatttcttttgtatactccctaaacacacagagtttactgggtcagatttaactgtgagcatttatatgcctacttccaggcatcgtcatctgatgtttcactgctactggtttcggtgtctgagtcctcaaactctgctttgcaagtgcttctccaaggggagaacagactggaactgcggctctgcaagaagccattctttccaaagccatttcttctcagctgctctgtcttcatgtggaactctttgagctcatcctctgtgaggggaaggcaattctcatcattttcaggatattcctgccaacccatagctttcaataacctgtgctctgcttctagagagtgtgagagaacctccccttcttccactacagggagggcaagaccattttgatgacagccttcctccccattttcctttggttcaggtgtgctgttgtcctccaaatcttccagcttgtcacagtctctattctctgagaagtctccattccggtcatccttcagagttttcaggaactcactcttcctgtcggtggttcggcgggtcaacttggtcagacgagaggagctgatctcaattggaggggtggtgctggagggactctctttgggagaactcagagctgcaccactagccagtaccactggtttggtaacagagattggactggtaaaagcagactcccggctagaggaaagggatcctgacttgtgctccatcctgttagctttccatgcattaggcttggaaggaggtggtacaggcttaggaaccaggttcttatagacacttggaaccacggatgacaatttgttcccatttgcatggtgagatcctggtgaggtgaatgcagcagagaaggcagcagcaggatcctctttggaaacttttttgataactagcatcttggagggttgcttggcactaggcgggttttcccatactccagaaggtgtcccaataggtctgcatggctgatgctgtttgccagcttctggattcaaggaaggaaagtcctcctcttcaaactgcaacttttccaccttgtcttctttcttttcttccctaatctccataggtggcttttcctgaaaagcacaccctttccgggagtggaagctgccattccaatggcgatggttccctgtgccacctccactacgttggctcatgccatcatgacctcgggaagagctatgccaaccagatgggttccctgtgattccagcatatgctcccttagagacaccagagtccacagaatcatggcggaacagggagggctggtgccaagaatctcctgcagttcgtaggggaccattgttaaaaaaaccatcagaggaattatgtcgacggcggcttactccaaatctaccttctcctctgggtaggtgctctccgtgtttttcgaaggtggcagtaggtgacttagctgactgtggtgttgagaaatttagccaagcaggaacaaaatcatgctgcgccatttaggtccagtgtctcctttcagtaaggtgaggcatccaacctcatggccaggatcccagagtgtaacctctgtggtcctgtttctgaactcgagtcggccagctggatctcccacaaggtttccttgttaaaagggtgcttaagtaacctggccggcagcacgacttatgatgaagcacgaagaagccaggttctgtgtcgatcactctctcagtcccctcaactgctcatcttaaactatttggttcctgacacgtttccaaaaggggaaaggggaaaaggggaaggggggaaggggaacataaaaagtatttgttacatttaaaaagggggggaaggggaaagagctgtatctatgttcacctcattcaacttccttgagttatggcactatgatgttgcttaattaggtaagacatggatatttgcaccgagtgcaaatactgttcataacaaggtcatagctagaaagacagatgggctcaagtgtggacaaataatgtcatcaaggtaatagatcaaaaatattaaagccctataaaagatctgagcagtcaactccaaaacatccacatgacaaagtccttaaaatacaaatctcattactcttactcatgcaactgctaaaaaatagtgtgcagatatgtatttatatttgccttaaccttcaaaatctagggacataaatcttgtctttgttaaaaaaaaataaaaaataaaaatagacaggaatttgctacacttttccctccacgaacagcagctttcaaggcaaatttcttggtataaagctactaaatgtatattctatgtctttggcctttactatttataaattcagagcaaagttaaaacattagaacgatgggtaggatggatattaagaaatagtcaaggagaaatataggtccaaaatgaggatttcttctcttcagttttctgtgtttcacttgttctgctccttcccaaaatctaaattgagccactggaaggagatatgaagaatcttctatgctttggtagagaagtcacttattattttggatccatttccaccacttcacaatcatttgaaaggccacacgaatctatcactctctacaaggacttgcaaaccggtttcggaggaacgtgtgttttccggccctttcccaccttccgctccttacttctcgtgtgcgcgtcgttgagactccagtccccagc

SEQ ID NO: 18754 - RNA, 2938 nt, Homo sapiens
  source 1..2938: mol_type = other RNA
tgagtgtgtgtgtgtgagtgtgtttaaaaaatctgtcccaccacacaaacttctctctataaagcagataacagggaagaacaataacaaaagcaaaacaagccaattgctctctctttgggatatgattatttcccttgtgaatgaagtattcaacaacataagaaaaggaaaagaacgatttcttttgtatactccctaaacacacagagtttactgggtcagatttaactgtgagcatttatatgcctacttccaggcatcgtcatctgatgtttcactgctactggtttcggtgtctgagtcctcaaactctgctttgcaagtgcttctccaaggggagaacagactggaactgcggctctgcaagaagccattctttccaaagccatttcttctcagctgctctgtcttcatgtggaactctttgagctcatcctctgtgaggggaaggcaattctcatcattttcaggatattcctgccaacccatagctttcaataacctgtgctctgcttctagagagtgtgagagaacctccccttcttccactacagggagggcaagaccattttgatgacagccttcctccccattttcctttggttcaggtgtgctgttgtcctccaaatcttccagcttgtcacagtctctattctctgagaagtctccattccggtcatccttcagagttttcaggaactcactcttcctgtcggtggttcggcgggtcaacttggtcagacgagaggagctgatctcaattggaggggtggtgctggagggactctctttgggagaactcagagctgcaccactagccagtaccactggtttggtaacagagattggactggtaaaagcagactcccggctagaggaaagggatcctgacttgtgctccatcctgttagctttccatgcattaggcttggaaggaggtggtacaggcttaggaaccaggttcttatagacacttggaaccacggatgacaatttgttcccatttgcatggtgagatcctggtgaggtgaatgcagcagagaaggcagcagcaggatcctctttggaaacttttttgataactagcatcttggagggttgcttggcactaggcgggttttcccatactccagaaggtgtcccaataggtctgcatggctgatgctgtttgccagcttctggattcaaggaaggaaagtcctcctcttcaaactgcaacttttccaccttgtcttctttcttttcttccctaatctccataggtggcttttcctgaaaagcacaccctttccgggagtggaagctgccattccaatggcgatggttccctgtgccacctccactacgttggctcatgccatcatgacctcgggaagagctatgccaaccagatgggttccctgtgattccagcatatgctcccttagagacaccagagtccacagaatcatggcggaacagggagggctggtgccaagaatctcctgcagttcgtaggggaccattgttaaaaaaaccatcagaggaattatgtcgacggcggcttactccaaatctaccttctcctctgggtaggtgctctccgtgtttttcgaaggtggcagtaggtgacttagctgactgtggtgttgagaaatttagccaagcaggaacaaaatcatgctgcgccatttaggtccagtgtctcctttcagtaaggtgaggcatccaacctcatggccaggatcccagagtgtaacctctgtggtcctgtttctgaactcgagtcggccagctggatctcccacaaggtttccttgttaaaagggtgcttaagtaacctggccggcagcacgacttatgatgaagcacgaagaagccaggttctgtgtcgatcactctctcagtcccctcaactgctcatcttaaactatttggttcctgacacgtttccaaaaggggaaaggggaaaaggggaaggggggaaggggaacataaaaagtatttgttacatttaaaaagggggggaaggggaaagagctgtatctatgttcacctcattcaacttccttgagttatggcactatgatgttgcttaattaggtaagacatggatatttgcaccgagtgcaaatactgttcataacaaggtcatagctagaaagacagatgggctcaagtgtggacaaataatgtcatcaaggtaatagatcaaaaatattaaagccctataaaagatctgagcagtcaactccaaaacatccacatgacaaagtccttaaaatacaaatctcattactcttactcatgcaactgctaaaaaatagtgtgcagatatgtatttatatttgccttaaccttcaaaatctagggacataaatcttgtctttgttaaaaaaaaataaaaaataaaaatagacaggaatttgctacacttttccctccacgaacagcagctttcaaggcaaatttcttggtataaagctactaaatgtatattctatgtctttggcctttactatttataaattcagagcaaagttaaaacattagaacgatgggtaggatggatattaagaaatagtcaaggagaaatataggtccaaaatgaggatttcttctcttcagttttctgtgtttcacttgttctgctccttcccaaaatctaaattgagccactggaaggagatatgaagaatcttctatgctttggtagagaagtcacttattattttggatccatttccaccacttcacaatcatttgaaaggccacacgaatctatcactctttgttttcacccagcataaggagagttaaaggtgagacaccaacgggcagcggcggagctatggccagggactagacgctgcgtctgaggacgcgtccccagcttgtcgacccggcagaggcggctagtccacaaccataacaaagctcttcccaaaatggctgc

SEQ ID NO: 18755 - RNA, 2926 nt, Homo sapiens
  source 1..2926: mol_type = other RNA
tgagtgtgtgtgtgtgagtgtgtttaaaaaatctgtcccaccacacaaacttctctctataaagcagataacagggaagaacaataacaaaagcaaaacaagccaattgctctctctttgggatatgattatttcccttgtgaatgaagtattcaacaacataagaaaaggaaaagaacgatttcttttgtatactccctaaacacacagagtttactgggtcagatttaactgtgagcatttatatgcctacttccaggcatcgtcatctgatgtttcactgctactggtttcggtgtctgagtcctcaaactctgctttgcaagtgcttctccaaggggagaacagactggaactgcggctctgcaagaagccattctttccaaagccatttcttctcagctgctctgtcttcatgtggaactctttgagctcatcctctgtgaggggaaggcaattctcatcattttcaggatattcctgccaacccatagctttcaataacctgtgctctgcttctagagagtgtgagagaacctccccttcttccactacagggagggcaagaccattttgatgacagccttcctccccattttcctttggttcaggtgtgctgttgtcctccaaatcttccagcttgtcacagtctctattctctgagaagtctccattccggtcatccttcagagttttcaggaactcactcttcctgtcggtggttcggcgggtcaacttggtcagacgagaggagctgatctcaattggaggggtggtgctggagggactctctttgggagaactcagagctgcaccactagccagtaccactggtttggtaacagagattggactggtaaaagcagactcccggctagaggaaagggatcctgacttgtgctccatcctgttagctttccatgcattaggcttggaaggaggtggtacaggcttaggaaccaggttcttatagacacttggaaccacggatgacaatttgttcccatttgcatggtgagatcctggtgaggtgaatgcagcagagaaggcagcagcaggatcctctttggaaacttttttgataactagcatcttggagggttgcttggcactaggcgggttttcccatactccagaaggtgtcccaataggtctgcatggctgatgctgtttgccagcttctggattcaaggaaggaaagtcctcctcttcaaactgcaacttttccaccttgtcttctttcttttcttccctaatctccataggtggcttttcctgaaaagcacaccctttccgggagtggaagctgccattccaatggcgatggttccctgtgccacctccactacgttggctcatgccatcatgacctcgggaagagctatgccaaccagatgggttccctgtgattccagcatatgctcccttagagacaccagagtccacagaatcatggcggaacagggagggctggtgccaagaatctcctgcagttcgtaggggaccattgttaaaaaaaccatcagaggaattatgtcgacggcggcttactccaaatctaccttctcctctgggtaggtgctctccgtgtttttcgaaggtggcagtaggtgacttagctgactgtggtgttgagaaatttagccaagcaggaacaaaatcatgctgcgccatttaggtccagtgtctcctttcagtaaggtgaggcatccaacctcatggccaggatcccagagtgtaacctctgtggtcctgtttctgaactcgagtcggccagctggatctcccacaaggtttccttgttaaaagggtgcttaagtaacctggccggcagcacgacttatgatgaagcacgaagaagccaggttctgtgtcgatcactctctcagtcccctcaactgctcatcttaaactatttggttcctgacacgtttccaaaaggggaaaggggaaaaggggaaggggggaaggggaacataaaaagtatttgttacatttaaaaagggggggaaggggaaagagctgtatctatgttcacctcattcaacttccttgagttatggcactatgatgttgcttaattaggtaagacatggatatttgcaccgagtgcaaatactgttcataacaaggtcatagctagaaagacagatgggctcaagtgtggacaaataatgtcatcaaggtaatagatcaaaaatattaaagccctataaaagatctgagcagtcaactccaaaacatccacatgacaaagtccttaaaatacaaatctcattactcttactcatgcaactgctaaaaaatagtgtgcagatatgtatttatatttgccttaaccttcaaaatctagggacataaatcttgtctttgttaaaaaaaaataaaaaataaaaatagacaggaatttgctacacttttccctccacgaacagcagctttcaaggcaaatttcttggtataaagctactaaatgtatattctatgtctttggcctttactatttataaattcagagcaaagttaaaacattagaacgatgggtaggatggatattaagaaatagtcaaggagaaatataggtccaaaatgaggatttcttctcttcagttttctgtgtttcacttgttctgctccttcccaaaatctaaattgagccactggaaggagatatgaagaatcttctatgctttggtagagaagtcacttattattttggatccatttccaccacttcacaatcatttgaaaggccacacgaatctatcactctttgttttcacccagcataaggagagttaaaggtgagacaccaactctacaaggacttgcaaaccggtttcggaggaacgtgtgttttccggccctttcccaccttccgctccttacttctcgtgtgcgcgtcgttgagactccagtccccagc

SEQ ID NO: 18756 - RNA, 2930 nt, Homo sapiens
  source 1..2930: mol_type = other RNA
tgagtgtgtgtgtgtgagtgtgtttaaaaaatctgtcccaccacacaaacttctctctataaagcagataacagggaagaacaataacaaaagcaaaacaagccaattgctctctctttgggatatgattatttcccttgtgaatgaagtattcaacaacataagaaaaggaaaagaacgatttcttttgtatactccctaaacacacagagtttactgggtcagatttaactgtgagcatttatatgcctacttccaggcatcgtcatctgatgtttcactgctactggtttcggtgtctgagtcctcaaactctgctttgcaagtgcttctccaaggggagaacagactggaactgcggctctgcaagaagccattctttccaaagccatttcttctcagctgctctgtcttcatgtggaactctttgagctcatcctctgtgaggggaaggcaattctcatcattttcaggatattcctgccaacccatagctttcaataacctgtgctctgcttctagagagtgtgagagaacctccccttcttccactacagggagggcaagaccattttgatgacagccttcctccccattttcctttggttcaggtgtgctgttgtcctccaaatcttccagcttgtcacagtctctattctctgagaagtctccattccggtcatccttcagagttttcaggaactcactcttcctgtcggtggttcggcgggtcaacttggtcagacgagaggagctgatctcaattggaggggtggtgctggagggactctgggcaaataccacaaacaggttgctcctctttgggagaactcagagctgcaccactagccagtaccactggtttggtaacagagattggactggtaaaagcagactcccggctagaggaaagggatcctgacttgtgctccatcctgttagctttccatgcattaggcttggaaggaggtggtacaggcttaggaaccaggttcttatagacacttggaaccacggatgacaatttgttcccatttgcatggtgagatcctggtgaggtgaatgcagcagagaaggcagcagcaggatcctctttggaaacttttttgataactagcatcttggagggttgcttggcactaggcgggttttcccatactccagaaggtgtcccaataggtctgcatggctgatgctgtttgccagcttctggattcaaggaaggaaagtcctcctcttcaaactgcaacttttccaccttgtcttctttcttttcttccctaatctccataggtggcttttcctgaaaagcacaccctttccgggagtggaagctgccattccaatggcgatggttccctgtgccacctccactacgttggctcatgccatcatgacctcgggaagagctatgccaaccagatgggttccctgtgattccagcatatgctcccttagagacaccagagtccacagaatcatggcggaacagggagggctggtgccaagaatctcctgcagttcgtaggggaccattgttaaaaaaaccatcagaggaattatgtcgacggcggcttactccaaatctaccttctcctctgggtaggtgctctccgtgtttttcgaaggtggcagtaggtgacttagctgactgtggtgttgagaaatttagccaagcaggaacaaaatcatgctgcgccatttaggtccagtgtctcctttcagtaaggtgaggcatccaacctcatggccaggatcccagagtgtaacctctgtggtcctgtttctgaactcgagtcggccagctggatctcccacaaggtttccttgttaaaagggtgcttaagtaacctggccggcagcacgacttatgatgaagcacgaagaagccaggttctgtgtcgatcactctctcagtcccctcaactgctcatcttaaactatttggttcctgacacgtttccaaaaggggaaaggggaaaaggggaaggggggaaggggaacataaaaagtatttgttacatttaaaaagggggggaaggggaaagagctgtatctatgttcacctcattcaacttccttgagttatggcactatgatgttgcttaattaggtaagacatggatatttgcaccgagtgcaaatactgttcataacaaggtcatagctagaaagacagatgggctcaagtgtggacaaataatgtcatcaaggtaatagatcaaaaatattaaagccctataaaagatctgagcagtcaactccaaaacatccacatgacaaagtccttaaaatacaaatctcattactcttactcatgcaactgctaaaaaatagtgtgcagatatgtatttatatttgccttaaccttcaaaatctagggacataaatcttgtctttgttaaaaaaaaataaaaaataaaaatagacaggaatttgctacacttttccctccacgaacagcagctttcaaggcaaatttcttggtataaagctactaaatgtatattctatgtctttggcctttactatttataaattcagagcaaagttaaaacattagaacgatgggtaggatggatattaagaaatagtcaaggagaaatataggtccaaaatgaggatttcttctcttcagttttctgtgtttcacttgttctgctccttcccaaaatctaaattgagccactggaaggagatatgaagaatcttctatgctttggtagagaagtcacttattattttggatccatttccaccacttcacaatcatttgaaaggccacacgaatctatcactcgggcagcggcggagctatggccagggactagacgctgcgtctgaggacgcgtccccagcttgtcgacccggcagaggcggctagtccacaaccataacaaagctcttcccaaaatggctgcccggcccac

SEQ ID NO: 18757 - RNA, 2966 nt, Homo sapiens
  source 1..2966: mol_type = other RNA
tgagtgtgtgtgtgtgagtgtgtttaaaaaatctgtcccaccacacaaacttctctctataaagcagataacagggaagaacaataacaaaagcaaaacaagccaattgctctctctttgggatatgattatttcccttgtgaatgaagtattcaacaacataagaaaaggaaaagaacgatttcttttgtatactccctaaacacacagagtttactgggtcagatttaactgtgagcatttatatgcctacttccaggcatcgtcatctgatgtttcactgctactggtttcggtgtctgagtcctcaaactctgctttgcaagtgcttctccaaggggagaacagactggaactgcggctctgcaagaagccattctttccaaagccatttcttctcagctgctctgtcttcatgtggaactctttgagctcatcctctgtgaggggaaggcaattctcatcattttcaggatattcctgccaacccatagctttcaataacctgtgctctgcttctagagagtgtgagagaacctccccttcttccactacagggagggcaagaccattttgatgacagccttcctccccattttcctttggttcaggtgtgctgttgtcctccaaatcttccagcttgtcacagtctctattctctgagaagtctccattccggtcatccttcagagttttcaggaactcactcttcctgtcggtggttcggcgggtcaacttggtcagacgagaggagctgatctcaattggaggggtggtgctggagggactctgggcaaataccacaaacaggttgctcctctttgggagaactcagagctgcaccactagccagtaccactggtttggtaacagagattggactggtaaaagcagactcccggctagaggaaagggatcctgacttgtgctccatcctgttagctttccatgcattaggcttggaaggaggtggtacaggcttaggaaccaggttcttatagacacttggaaccacggatgacaatttgttcccatttgcatggtgagatcctggtgaggtgaatgcagcagagaaggcagcagcaggatcctctttggaaacttttttgataactagcatcttggagggttgcttggcactaggcgggttttcccatactccagaaggtgtcccaataggtctgcatggctgatgctgtttgccagcttctggattcaaggaaggaaagtcctcctcttcaaactgcaacttttccaccttgtcttctttcttttcttccctaatctccataggtggcttttcctgaaaagcacaccctttccgggagtggaagctgccattccaatggcgatggttccctgtgccacctccactacgttggctcatgccatcatgacctcgggaagagctatgccaaccagatgggttccctgtgattccagcatatgctcccttagagacaccagagtccacagaatcatggcggaacagggagggctggtgccaagaatctcctgcagttcgtaggggaccattgttaaaaaaaccatcagaggaattatgtcgacggcggcttactccaaatctaccttctcctctgggtaggtgctctccgtgtttttcgaaggtggcagtaggtgacttagctgactgtggtgttgagaaatttagccaagcaggaacaaaatcatgctgcgccatttaggtccagtgtctcctttcagtaaggtgaggcatccaacctcatggccaggatcccagagtgtaacctctgtggtcctgtttctgaactcgagtcggccagctggatctcccacaaggtttccttgttaaaagggtgcttaagtaacctggccggcagcacgacttatgatgaagcacgaagaagccaggttctgtgtcgatcactctctcagtcccctcaactgctcatcttaaactatttggttcctgacacgtttccaaaaggggaaaggggaaaaggggaaggggggaaggggaacataaaaagtatttgttacatttaaaaagggggggaaggggaaagagctgtatctatgttcacctcattcaacttccttgagttatggcactatgatgttgcttaattaggtaagacatggatatttgcaccgagtgcaaatactgttcataacaaggtcatagctagaaagacagatgggctcaagtgtggacaaataatgtcatcaaggtaatagatcaaaaatattaaagccctataaaagatctgagcagtcaactccaaaacatccacatgacaaagtccttaaaatacaaatctcattactcttactcatgcaactgctaaaaaatagtgtgcagatatgtatttatatttgccttaaccttcaaaatctagggacataaatcttgtctttgttaaaaaaaaataaaaaataaaaatagacaggaatttgctacacttttccctccacgaacagcagctttcaaggcaaatttcttggtataaagctactaaatgtatattctatgtctttggcctttactatttataaattcagagcaaagttaaaacattagaacgatgggtaggatggatattaagaaatagtcaaggagaaatataggtccaaaatgaggatttcttctcttcagttttctgtgtttcacttgttctgctccttcccaaaatctaaattgagccactggaaggagatatgaagaatcttctatgctttggtagagaagtcacttattattttggatccatttccaccacttcacaatcatttgaaaggccacacgaatctatcactctttgttttcacccagcataaggagagttaaaggtgagacaccaacgggcagcggcggagctatggccagggactagacgctgcgtctgaggacgcgtccccagcttgtcgacccggcagaggcggctagtccacaaccataacaaagctcttcccaaaatggctgc

SEQ ID NO: 18758 - RNA, 2779 nt, Homo sapiens
  source 1..2779: mol_type = other RNA
tgagtgtgtgtgtgtgagtgtgtttaaaaaatctgtcccaccacacaaacttctctctataaagcagataacagggaagaacaataacaaaagcaaaacaagccaattgctctctctttgggatatgattatttcccttgtgaatgaagtattcaacaacataagaaaaggaaaagaacgatttcttttgtatactccctaaacacacagagtttactgggtcagatttaactgtgagcatttatatgcctacttccaggcatcgtcatctgatgtttcactgctactggtttcggtgtctgagtcctcaaactctgctttgcaagtgcttctccaaggggagaacagactggaactgcggctctgcaagaagccattctttccaaagccatttcttctcagctgctctgtcttcatgtggaactctttgagctcatcctctgtgaggggaaggcaattctcatcattttcaggatattcctgccaacccatagctttcaataacctgtgctctgcttctagagagtgtgagagaacctccccttcttccactacagggagggcaagaccattttgatgacagccttcctccccattttcctttggttcaggtgtgctgttgtcctccaactctttgggagaactcagagctgcaccactagccagtaccactggtttggtaacagagattggactggtaaaagcagactcccggctagaggaaagggatcctgacttgtgctccatcctgttagctttccatgcattaggcttggaaggaggtggtacaggcttaggaaccaggttcttatagacacttggaaccacggatgacaatttgttcccatttgcatggtgagatcctggtgaggtgaatgcagcagagaaggcagcagcaggatcctctttggaaacttttttgataactagcatcttggagggttgcttggcactaggcgggttttcccatactccagaaggtgtcccaataggtctgcatggctgatgctgtttgccagcttctggattcaaggaaggaaagtcctcctcttcaaactgcaacttttccaccttgtcttctttcttttcttccctaatctccataggtggcttttcctgaaaagcacaccctttccgggagtggaagctgccattccaatggcgatggttccctgtgccacctccactacgttggctcatgccatcatgacctcgggaagagctatgccaaccagatgggttccctgtgattccagcatatgctcccttagagacaccagagtccacagaatcatggcggaacagggagggctggtgccaagaatctcctgcagttcgtaggggaccattgttaaaaaaaccatcagaggaattatgtcgacggcggcttactccaaatctaccttctcctctgggtaggtgctctccgtgtttttcgaaggtggcagtaggtgacttagctgactgtggtgttgagaaatttagccaagcaggaacaaaatcatgctgcgccatttaggtccagtgtctcctttcagtaaggtgaggcatccaacctcatggccaggatcccagagtgtaacctctgtggtcctgtttctgaactcgagtcggccagctggatctcccacaaggtttccttgttaaaagggtgcttaagtaacctggccggcagcacgacttatgatgaagcacgaagaagccaggttctgtgtcgatcactctctcagtcccctcaactgctcatcttaaactatttggttcctgacacgtttccaaaaggggaaaggggaaaaggggaaggggggaaggggaacataaaaagtatttgttacatttaaaaagggggggaaggggaaagagctgtatctatgttcacctcattcaacttccttgagttatggcactatgatgttgcttaattaggtaagacatggatatttgcaccgagtgcaaatactgttcataacaaggtcatagctagaaagacagatgggctcaagtgtggacaaataatgtcatcaaggtaatagatcaaaaatattaaagccctataaaagatctgagcagtcaactccaaaacatccacatgacaaagtccttaaaatacaaatctcattactcttactcatgcaactgctaaaaaatagtgtgcagatatgtatttatatttgccttaaccttcaaaatctagggacataaatcttgtctttgttaaaaaaaaataaaaaataaaaatagacaggaatttgctacacttttccctccacgaacagcagctttcaaggcaaatttcttggtataaagctactaaatgtatattctatgtctttggcctttactatttataaattcagagcaaagttaaaacattagaacgatgggtaggatggatattaagaaatagtcaaggagaaatataggtccaaaatgaggatttcttctcttcagttttctgtgtttcacttgttctgctccttcccaaaatctaaattgagccactggaaggagatatgaagaatcttctatgctttggtagagaagtcacttattattttggatccatttccaccacttcacaatcatttgaaaggccacacgaatctatcactctttgttttcacccagcataaggagagttaaaggtgagacaccaacgggcagcggcggagctatggccagggactagacgctgcgtctgaggacgcgtccccagcttgtcgacccggcagaggcggctagtccacaaccataacaaagctcttcccaaaatggctgc

SEQ ID NO: 18759 - RNA, 4206 nt, Homo sapiens
  source 1..4206: mol_type = other RNA
tgagtgtgtgtgtgtgagtgtgtttaaaggaaccacaaagcaaagataaggtttctctttttttcagagttcatgatcctaagactttctgtgttctctcctgtgactgagctgagtggggcttgtttgtttctcttctgtaaacaaggatattgttttttcccttttaggagtagagtcatcatttcaatcacatgaaagaaactagcttctccctgtgtccgtctggtccggagagcttgcgttttaggaacgtggtaacgtagtagctgaaaggagccaacggcttgatgggatagtctgtgccgaaactcccgatcccaacatgctgcgtacagacacacgagcgaaaacggttcgccctcccctgggtatccaaggatgaggacgtgagtatgaaagtggtccccgggcccagtatccattccgtcgtgtgacagacaggctaactgaccatcccttctccaataccaaaacattcttttttgttgttggggttggttgcttttttttttttttttaaatcgtttttctttttctttttttttttttaataagttaaagttaatacaaatataaaaaggggaaagtcctctagattcaatgacatccacaaattgtacattatttacaccaaaagcacagggctcgtgtgggtgaacagtctgcagtcaaagccgatgctgggtgtcctgtagtgtagcagcccccgcgccgggggctcaggctcaactgagggttttgtcattttcaagtctgaaagtggctgttctcctgcctttgttgtttcttcttttcctggcgtctgggtttttctcccaatggggtgggtggtttgtgtcccgattcactgctagtcccagaaggtgtccagccgagactctttcgggaggaggctcttcgtgctggtactggtgttgtgatcggaacgtgtcgatcccctcttctcatcactgctgctccaactggatttattactccgggaatggtacttctgggcggggtagttggggtgcggctggtggtctgtggtggttggggcataggcaggttgcttgtcacaccttttgctaacagagccttggttggagcctaagagaatggaggagggcgtctctctggagccagaaaggtcaagggtcgagccactctccttgcttttctcagctgacgtctccttctctttggaggcgctggccgtttctgaaggtgctgattgtgtgctcgaggagctcccctgggaggacttatttagtgtttctgtgttcacctcagcatccgcttcctgctgaggagcagtagctgactgggtgcaggacttcatgtgctcaggccagtgggcttgctggcaggggtagtcacagtagctggtgttccaacagcagtaaaagatggcctccttcttgcagttggcgcaccactgcttcttcttggtctcatccaccgcctgctgcttctccaactccagctgcttcttcacctcggcgatgagccggtcccgctcctgctccaggctctgccgcatctccgccatggtcagctctaagttgtgtttcatttcggagagctcttgctggtgcagccactggagcttctctatctcgatcctcagcctgcgaatctcagctattgtgcttccagtagtgtttttagaaagatcgttgtatatttctgtcattgttccttttattgcatccatcattttgctagtgtacttggcaatatcagcggcgacatcagctgaggcagtggcgatgggcaggtcagcgttgactgaggacacaagggtgctcatggaccccgagctggtgaccaggggcgatgactgtgtgctggtcaccagggtgatggtggacgtggatgggctctgtgtgatctccttctgctggacagcatcctgtttgggagatggttctttgggttccttcttattttttcgaccctcccgcccagaatggtcttctcctaaatctatgacaagttcgctctctgaatcagagtccaggcccaaatggactgttggggaatccgtctcatcttttcccttcagtttatcctttatggggtgaggtgaaggttttgccttttcggaaaagtccttctcaggctcagggctggccttgtccttgactgctccagggtctgccttctcgctggctggtgacgtgcttttcagctcctctttaatctccactgggtttgtaggcttgggcttttttttaacagcagatggctctttgtccatctgacaaccttctttgtcctctgtgtcttctggctcgttcttagacttctgctcatcatcactgatatactcactatcgctactatctgacttctcagaatcctccgaatcgctgtgctctacggccgtatagacatcttccgagatttcatttatgcctaattgtgctttgcaactctctatggtcttgtcaagattcagctggaacctgctacgaatctggcgcttgggagagatgagaggaacaggggtggactgttgctggaccgactcgctcagctccttcaaatccatctcagctttgcttcgatccaggttaagattcaggatgctgccggtggtggaggttttgtccgttttcgtcgtgataggagctgacagttgaggagagaagggctttgggctgccggataaactccctgcttgtcccgtcttggtggaggctggtgaagctgtgctcttatccaggaagtccatggactcctcgctcgcactgaagtggctcgacgtggccttcttctcagcatcctgctccacgtcggagcccgtgtgcacagaagagtttgtgctcatgggggagcgcggcatatccgacaaggaaatccggcggcctgtgcccccactcagcacaggcttgctcatcaggatcttgggggatgccgtcatgtcaaagttgagcttgaccttctcctgcttgtctatcttggcagtgccggcgctggggttggtgggatcgagcagcatttgatactggctgttgggtgtgtagggtgtcctaaatggagagtaattaaaaaccccaaacttcctgcggatgttctccacgtaaacctccatctcttgcatggcactgttgaagatgctcttagtctttttcacagaaaaaggaatttctttagacatgaggtagcaattatttattggaacccaggccctgtcatgttgtccaaagaatcgggcatcgacctgcccgtctttatcccttagagcttttgcaggccagaatggaaaccccttcagtttggcccagaccaaaggatgtggattgctacaaggctcacaaaaccagttatctcgtttttggcaagcagctagataacattctggacatacttcgatttcattcatctcatgttcacagattttgatgactactttcgctatttgcgtcaatttgtgatttcccccattataaatgatgcagttgtgcaaaatccactttgcatcagccaggaaggcttctgtgcagccatacattttctttttcgcattcttttccaatgtacaaaggtccattggatggaagatgtattccgcatagtcagggtgctgttccaatggaacgggcttctggaatgcatctgtccctggctgtttcattttctgaatggcaaacttgagcaggtaggataactgttcaatggtgagcattgtcatggctttactctgggtctcgatgcattctgctactgtaattttctcacattcaggacaaaaccagtccccctctggttccgatgtcagtctcagacacttagcgtgataaacccggggacagagctcacagcaaaggacttggccttcccggtgacaaacccagcagtagaaatcattccgtccatcctgcggtacaacatcaacagggtctgtggtgagtggctgcttcatatagtaaaacggaccatgtcttagttctgactgctccttattgttactgttcagtaagccaggtttctttttctttttaatggggcttgttgatgtgtcctgcggcgagtggccattggaagaatgtggagggctggggaactttcttttctgggctgttctctctgcagagccaggatctttggagcgagtagagatatccatgccctctaccacctcctgttctgtttttatttcctcttcagccaagctctgtggatgcattgttaacactgtgtaatgtcaatacttat

SEQ ID NO: 18760 - RNA, 4601 nt, Homo sapiens
  source 1..4601: mol_type = other RNA
tgagtgtgtgtgtgtgagtgtgtttaaaggaaccacaaagcaaagataaggtttctctttttttcagagttcatgatcctaagactttctgtgttctctcctgtgactgagctgagtggggcttgtttgtttctcttctgtaaacaaggatattgttttttcccttttaggagtagagtcatcatttcaatcacatgaaagaaactagcttctccctgtgtccgtctggtccggagagcttgcgttttaggaacgtggtaacgtagtagctgaaaggagccaacggcttgatgggatagtctgtgccgaaactcccgatcccaacatgctgcgtacagacacacgagcgaaaacggttcgccctcccctgggtatccaaggatgaggacgtgagtatgaaagtggtccccgggcccagtatccattccgtcgtgtgacagacaggctaactgaccatcccttctccaataccaaaacattcttttttgttgttggggttggttgcttttttttttttttttaaatcgtttttctttttctttttttttttttaataagttaaagttaatacaaatataaaaaggggaaagtcctctagattcaatgacatccacaaattgtacattatttacaccaaaagcacagggctcgtgtgggtgaacagtctgcagtcaaagccgatgctgggtgtcctgtagtgtagcagcccccgcgccgggggctcaggctcaactgagggttttgtcattttcaagtctgaaagtggctgttctcctgcctttgttgtttcttcttttcctggcgtctgggtttttctcccaatggggtgggtggtttgtgtcccgattcactgctagtcccagaaggtgtccagccgagactctttcgggaggaggctcttcgtgctggtactggtgttgtgatcggaacgtgtcgatcccctcttctcatcactgctgctccaactggatttattactccgggaatggtacttctgggcggggtagttggggtgcggctggtggtctgtggtggttggggcataggcaggttgcttgtcacaccttttgctaacagagccttggttggagcctaagagaatggaggagggcgtctctctggagccagaaaggtcaagggtcgagccactctccttgcttttctcagctgacgtctccttctctttggaggcgctggccgtttctgaaggtgctgattgtgtgctcgaggagctcccctgggaggacttatttagtgtttctgtgttcacctcagcatccgcttcctgctgaggagcagtagctgactgggtgcaggacttcatgtgctcaggccagtgggcttgctggcaggggtagtcacagtagctggtgttccaacagcagtaaaagatggcctccttcttgcagttggcgcaccactgcttcttcttggtctcatccaccgcctgctgcttctccaactccagctgcttcttcacctcggcgatgagccggtcccgctcctgctccaggctctgccgcatctccgccatggtcagctctaagttgtgtttcatttcggagagctcttgctggtgcagccactggagcttctctatctcgatcctcagcctgcgaatctcagctattgtgcttccagtagtgtttttagaaagatcgttgtatatttctgtcattgttccttttattgcatccatcattttgctagtgtacttggcaatatcagcggcgacatcagctgaggcagtggcgatgggcaggtcagcgttgactgaggacacaagggtgctcatggaccccgagctggtgaccaggggcgatgactgtgtgctggtcaccagggtgatggtggacgtggatgggctctgtgtgatctccttctgctggacagctttcacagcctgtctggtctgatatctcgtcccctgggaagactgaggctgctgctgctggttttgctgctgctgctgctgctgctgacgctgcatcttctgcatgtgccacttttgggaggacgtttgaaacttacttgatgagttccacacgacccgctgcacggccggggcagtctccttcggtaaaagcggcctctgctttttcactgggcttcctgtggcggcgggggccggggccgtgacggtgaccgtggaggacgtgctggtggtggctgtggcgccagccgcggaagtttgggcggaagagcgggtgagcaccggtgtttccgggggagaatggctgcccaccgtcgtggatggtggagttttacctacaacatcctgtttgggagatggttctttgggttccttcttattttttcgaccctcccgcccagaatggtcttctcctaaatctatgacaagttcgctctctgaatcagagtccaggcccaaatggactgttggggaatccgtctcatcttttcccttcagtttatcctttatggggtgaggtgaaggttttgccttttcggaaaagtccttctcaggctcagggctggccttgtccttgactgctccagggtctgccttctcgctggctggtgacgtgcttttcagctcctctttaatctccactgggtttgtaggcttgggcttttttttaacagcagatggctctttgtccatctgacaaccttctttgtcctctgtgtcttctggctcgttcttagacttctgctcatcatcactgatatactcactatcgctactatctgacttctcagaatcctccgaatcgctgtgctctacggccgtatagacatcttccgagatttcatttatgcctaattgtgctttgcaactctctatggtcttgtcaagattcagctggaacctgctacgaatctggcgcttgggagagatgagaggaacaggggtggactgttgctggaccgactcgctcagctccttcaaatccatctcagctttgcttcgatccaggttaagattcaggatgctgccggtggtggaggttttgtccgttttcgtcgtgataggagctgacagttgaggagagaagggctttgggctgccggataaactccctgcttgtcccgtcttggtggaggctggtgaagctgtgctcttatccaggaagtccatggactcctcgctcgcactgaagtggctcgacgtggccttcttctcagcatcctgctccacgtcggagcccgtgtgcacagaagagtttgtgctcatgggggagcgcggcatatccgacaaggaaatccggcggcctgtgcccccactcagcacaggcttgctcatcaggatcttgggggatgccgtcatgtcaaagttgagcttgaccttctcctgcttgtctatcttggcagtgccggcgctggggttggtgggatcgagcagcatttgatactggctgttgggtgtgtagggtgtcctaaatggagagtaattaaaaaccccaaacttcctgcggatgttctccacgtaaacctccatctcttgcatggcactgttgaagatgctcttagtctttttcacagaaaaaggaatttctttagacatgaggtagcaattatttattggaacccaggccctgtcatgttgtccaaagaatcgggcatcgacctgcccgtctttatcccttagagcttttgcaggccagaatggaaaccccttcagtttggcccagaccaaaggatgtggattgctacaaggctcacaaaaccagttatctcgtttttggcaagcagctagataacattctggacatacttcgatttcattcatctcatgttcacagattttgatgactactttcgctatttgcgtcaatttgtgatttcccccattataaatgatgcagttgtgcaaaatccactttgcatcagccaggaaggcttctgtgcagccatacattttctttttcgcattcttttccaatgtacaaaggtccattggatggaagatgtattccgcatagtcagggtgctgttccaatggaacgggcttctggaatgcatctgtccctggctgtttcattttctgaatggcaaacttgagcaggtaggataactgttcaatggtgagcattgtcatggctttactctgggtctcgatgcattctgctactgtaattttctcacattcaggacaaaaccagtccccctctggttccgatgtcagtctcagacacttagcgtgataaacccggggacagagctcacagcaaaggacttggccttcccggtgacaaacccagcagtagaaatcattccgtccatcctgcggtacaacatcaacagggtctgtggtgagtggctgcttcatatagtaaaacggaccatgtcttagttctgactgctccttattgttactgttcagtaagccaggtttctttttctttttaatggggcttgttgatgtgtcctgcggcgagtggccattggaagaatgtggagggctggggaactttcttttctgggctgttctctctgcagagccaggatctttggagcgagtagagatatccatgccctctaccacctcctgttctgtttttatttcctcttcagccaagcaggatctagcttcaaactcttccagaaacaccatgccctggtggaaggaaaggtgt

SEQ ID NO: 18761 - RNA, 4658 nt, Homo sapiens
  source 1..4658: mol_type = other RNA
tgagtgtgtgtgtgtgagtgtgtttaaaggaaccacaaagcaaagataaggtttctctttttttcagagttcatgatcctaagactttctgtgttctctcctgtgactgagctgagtggggcttgtttgtttctcttctgtaaacaaggatattgttttttcccttttaggagtagagtcatcatttcaatcacatgaaagaaactagcttctccctgtgtccgtctggtccggagagcttgcgttttaggaacgtggtaacgtagtagctgaaaggagccaacggcttgatgggatagtctgtgccgaaactcccgatcccaacatgctgcgtacagacacacgagcgaaaacggttcgccctcccctgggtatccaaggatgaggacgtgagtatgaaagtggtccccgggcccagtatccattccgtcgtgtgacagacaggctaactgaccatcccttctccaataccaaaacattcttttttgttgttggggttggttgcttttttttttttttttaaatcgtttttctttttctttttttttttttaataagttaaagttaatacaaatataaaaaggggaaagtcctctagattcaatgacatccacaaattgtacattatttacaccaaaagcacagggctcgtgtgggtgaacagtctgcagtcaaagccgatgctgggtgtcctgtagtgtagcagcccccgcgccgggggctcaggctcaactgagggttttgtcattttcaagtctgaaagtggctgttctcctgcctttgttgtttcttcttttcctggcgtctgggtttttctcccaatggggtgggtggtttgtgtcccgattcactgctagtcccagaaggtgtccagccgagactctttcgggaggaggctcttcgtgctggtactggtgttgtgatcggaacgtgtcgatcccctcttctcatcactgctgctccaactggatttattactccgggaatggtacttctgggcggggtagttggggtgcggctggtggtctgtggtggttggggcataggcaggttgcttgtcacaccttttgctaacagagccttggttggagcctaagagaatggaggagggcgtctctctggagccagaaaggtcaagggtcgagccactctccttgcttttctcagctgacgtctccttctctttggaggcgctggccgtttctgaaggtgctgattgtgtgctcgaggagctcccctgggaggacttatttagtgtttctgtgttcacctcagcatccgcttcctgctgaggagcagtagctgactgggtgcaggacttcatgtgctcaggccagtgggcttgctggcaggggtagtcacagtagctggtgttccaacagcagtaaaagatggcctccttcttgcagttggcgcaccactgcttcttcttggtctcatccaccgcctgctgcttctccaactccagctgcttcttcacctcggcgatgagccggtcccgctcctgctccaggctctgccgcatctccgccatggtcagctctaagttgtgtttcatttcggagagctcttgctggtgcagccactggagcttctctatctcgatcctcagcctgcgaatctcagctattgtgcttccagtagtgtttttagaaagatcgttgtatatttctgtcattgttccttttattgcatccatcattttgctagtgtacttggcaatatcagcggcgacatcagctgaggcagtggcgatgggcaggtcagcgttgactgaggacacaagggtgctcatggaccccgagctggtgaccaggggcgatgactgtgtgctggtcaccagggtgatggtggacgtggatgggctctgtgtgatctccttctgctggacagctttcacagcctgtctggtctgatatctcgtcccctgggaagactgaggctgctgctgctggttttgctgctgctgctgctgctgctgacgctgcatcttctgcatgtgccacttttgggaggacgtttgaaacttacttgatgagttccacacgacccgctgcacggccggggcagtctccttcggtaaaagcggcctctgctttttcactgggcttcctgtggcggcgggggccggggccgtgacggtgaccgtggaggacgtgctggtggtggctgtggcgccagccgcggaagtttgggcggaagagcgggtgagcaccggtgtttccgggggagaatggctgcccaccgtcgtggatggtggagttttacctacaacatcctgtttgggagatggttctttgggttccttcttattttttcgaccctcccgcccagaatggtcttctcctaaatctatgacaagttcgctctctgaatcagagtccaggcccaaatggactgttggggaatccgtctcatcttttcccttcagtttatcctttatggggtgaggtgaaggttttgccttttcggaaaagtccttctcaggctcagggctggccttgtccttgactgctccagggtctgccttctcgctggctggtgacgtgcttttcagctcctctttaatctccactgggtttgtaggcttgggcttttttttaacagcagatggctctttgtccatctgacaaccttctttgtcctctgtgtcttctggctcgttcttagacttctgctcatcatcactgatatactcactatcgctactatctgacttctcagaatcctccgaatcgctgtgctctacggccgtatagacatcttccgagatttcatttatgcctaattgtgctttgcaactctctatggtcttgtcaagattcagctggaacctgctacgaatctggcgcttgggagagatgagaggaacaggggtggactgttgctggaccgactcgctcagctccttcaaatccatctcagctttgcttcgatccaggttaagattcaggatgctgccggtggtggaggttttgtccgttttcgtcgtgataggagctgacagttgaggagagaagggctttgggctgccggataaactccctgcttgtcccgtcttggtggaggctggtgaagctgtgctcttatccaggaagtccatggactcctcgctcgcactgaagtggctcgacgtggccttcttctcagcatcctgctccacgtcggagcccgtgtgcacagaagagtttgtgctcatgggggagcgcggcatatccgacaaggaaatccggcggcctgtgcccccactcagcacaggcttgctcatcaggatcttgggggatgccgtcatgtcaaagttgagcttgaccttctcctgcttgtctatcttggcagtgccggcgctggggttggtgggatcgagcagcatttgatactggctgttgggtgtgtagggtgtcctaaatggagagtaattaaaaaccccaaacttcctgcggatgttctccacgtaaacctccatctcttgcatggcactgttgaagatgctcttagtctttttcacagaaaaaggaatttctttagacatgaggtagcaattatttattggaacccaggccctgtcatgttgtccaaagaatcgggcatcgacctgcccgtctttatcccttagagcttttgcaggccagaatggaaaccccttcagtttggcccagaccaaaggatgtggattgctacaaggctcacaaaaccagttatctcgtttttggcaagcagctagataacattctggacatacttcgatttcattcatctcatgttcacagattttgatgactactttcgctatttgcgtcaatttgtgatttcccccattataaatgatgcagttgtgcaaaatccactttgcatcagccaggaaggcttctgtgcagccatacattttctttttcgcattcttttccaatgtacaaaggtccattggatggaagatgtattccgcatagtcagggtgctgttccaatggaacgggcttctggaatgcatctgtccctggctgtttcattttctgaatggcaaacttgagcaggtaggataactgttcaatggtgagcattgtcatggctttactctgggtctcgatgcattctgctactgtaattttctcacattcaggacaaaaccagtccccctctggttccgatgtcagtctcagacacttagcgtgataaacccggggacagagctcacagcaaaggacttggccttcccggtgacaaacccagcagtagaaatcattccgtccatcctgcggtacaacatcaacagggtctgtggtgagtggctgcttcatatagtaaaacggaccatgtcttagttctgactgctccttattgttactgttcagtaagccaggtttctttttctttttaatggggcttgttgatgtgtcctgcggcgagtggccattggaagaatgtggagggctggggaactttcttttctgggctgttctctctgcagagccaggatctttggagcgagtagagatatccatgccctctaccacctcctgttctgtttttatttcctcttcagccaagccaacaaatgttcaagcaaccgtctcatttttccacagttaggaagagagaacaggctggcagatttgggactctgtggatgcattgttaacactgtgtaatgtcaatacttat

SEQ ID NO: 18762 - RNA, 4587 nt, Homo sapiens
  source 1..4587: mol_type = other RNA
tgagtgtgtgtgtgtgagtgtgtttaaaggaaccacaaagcaaagataaggtttctctttttttcagagttcatgatcctaagactttctgtgttctctcctgtgactgagctgagtggggcttgtttgtttctcttctgtaaacaaggatattgttttttcccttttaggagtagagtcatcatttcaatcacatgaaagaaactagcttctccctgtgtccgtctggtccggagagcttgcgttttaggaacgtggtaacgtagtagctgaaaggagccaacggcttgatgggatagtctgtgccgaaactcccgatcccaacatgctgcgtacagacacacgagcgaaaacggttcgccctcccctgggtatccaaggatgaggacgtgagtatgaaagtggtccccgggcccagtatccattccgtcgtgtgacagacaggctaactgaccatcccttctccaataccaaaacattcttttttgttgttggggttggttgcttttttttttttttttaaatcgtttttctttttctttttttttttttaataagttaaagttaatacaaatataaaaaggggaaagtcctctagattcaatgacatccacaaattgtacattatttacaccaaaagcacagggctcgtgtgggtgaacagtctgcagtcaaagccgatgctgggtgtcctgtagtgtagcagcccccgcgccgggggctcaggctcaactgagggttttgtcattttcaagtctgaaagtggctgttctcctgcctttgttgtttcttcttttcctggcgtctgggtttttctcccaatggggtgggtggtttgtgtcccgattcactgctagtcccagaaggtgtccagccgagactctttcgggaggaggctcttcgtgctggtactggtgttgtgatcggaacgtgtcgatcccctcttctcatcactgctgctccaactggatttattactccgggaatggtacttctgggcggggtagttggggtgcggctggtggtctgtggtggttggggcataggcaggttgcttgtcacaccttttgctaacagagccttggttggagcctaagagaatggaggagggcgtctctctggagccagaaaggtcaagggtcgagccactctccttgcttttctcagctgacgtctccttctctttggaggcgctggccgtttctgaaggtgctgattgtgtgctcgaggagctcccctgggaggacttatttagtgtttctgtgttcacctcagcatccgcttcctgctgaggagcagtagctgactgggtgcaggacttcatgtgctcaggccagtgggcttgctggcaggggtagtcacagtagctggtgttccaacagcagtaaaagatggcctccttcttgcagttggcgcaccactgcttcttcttggtctcatccaccgcctgctgcttctccaactccagctgcttcttcacctcggcgatgagccggtcccgctcctgctccaggctctgccgcatctccgccatggtcagctctaagttgtgtttcatttcggagagctcttgctggtgcagccactggagcttctctatctcgatcctcagcctgcgaatctcagctattgtgcttccagtagtgtttttagaaagatcgttgtatatttctgtcattgttccttttattgcatccatcattttgctagtgtacttggcaatatcagcggcgacatcagctgaggcagtggcgatgggcaggtcagcgttgactgaggacacaagggtgctcatggaccccgagctggtgaccaggggcgatgactgtgtgctggtcaccagggtgatggtggacgtggatgggctctgtgtgatctccttctgctggacagctttcacagcctgtctggtctgatatctcgtcccctgggaagactgaggctgctgctgctggttttgctgctgctgctgctgctgctgacgctgcatcttctgcatgtgccacttttgggaggacgtttgaaacttacttgatgagttccacacgacccgctgcacggccggggcagtctccttcggtaaaagcggcctctgctttttcactgggcttcctgtggcggcgggggccggggccgtgacggtgaccgtggaggacgtgctggtggtggctgtggcgccagccgcggaagtttgggcggaagagcgggtgagcaccggtgtttccgggggagaatggctgcccaccgtcgtggatggtggagttttacctacaacatcctgtttgggagatggttctttgggttccttcttattttttcgaccctcccgcccagaatggtcttctcctaaatctatgacaagttcgctctctgaatcagagtccaggcccaaatggactgttggggaatccgtctcatcttttcccttcagtttatcctttatggggtgaggtgaaggttttgccttttcggaaaagtccttctcaggctcagggctggccttgtccttgactgctccagggtctgccttctcgctggctggtgacgtgcttttcagctcctctttaatctccactgggtttgtaggcttgggcttttttttaacagcagatggctctttgtccatctgacaaccttctttgtcctctgtgtcttctggctcgttcttagacttctgctcatcatcactgatatactcactatcgctactatctgacttctcagaatcctccgaatcgctgtgctctacggccgtatagacatcttccgagatttcatttatgcctaattgtgctttgcaactctctatggtcttgtcaagattcagctggaacctgctacgaatctggcgcttgggagagatgagaggaacaggggtggactgttgctggaccgactcgctcagctccttcaaatccatctcagctttgcttcgatccaggttaagattcaggatgctgccggtggtggaggttttgtccgttttcgtcgtgataggagctgacagttgaggagagaagggctttgggctgccggataaactccctgcttgtcccgtcttggtggaggctggtgaagctgtgctcttatccaggaagtccatggactcctcgctcgcactgaagtggctcgacgtggccttcttctcagcatcctgctccacgtcggagcccgtgtgcacagaagagtttgtgctcatgggggagcgcggcatatccgacaaggaaatccggcggcctgtgcccccactcagcacaggcttgctcatcaggatcttgggggatgccgtcatgtcaaagttgagcttgaccttctcctgcttgtctatcttggcagtgccggcgctggggttggtgggatcgagcagcatttgatactggctgttgggtgtgtagggtgtcctaaatggagagtaattaaaaaccccaaacttcctgcggatgttctccacgtaaacctccatctcttgcatggcactgttgaagatgctcttagtctttttcacagaaaaaggaatttctttagacatgaggtagcaattatttattggaacccaggccctgtcatgttgtccaaagaatcgggcatcgacctgcccgtctttatcccttagagcttttgcaggccagaatggaaaccccttcagtttggcccagaccaaaggatgtggattgctacaaggctcacaaaaccagttatctcgtttttggcaagcagctagataacattctggacatacttcgatttcattcatctcatgttcacagattttgatgactactttcgctatttgcgtcaatttgtgatttcccccattataaatgatgcagttgtgcaaaatccactttgcatcagccaggaaggcttctgtgcagccatacattttctttttcgcattcttttccaatgtacaaaggtccattggatggaagatgtattccgcatagtcagggtgctgttccaatggaacgggcttctggaatgcatctgtccctggctgtttcattttctgaatggcaaacttgagcaggtaggataactgttcaatggtgagcattgtcatggctttactctgggtctcgatgcattctgctactgtaattttctcacattcaggacaaaaccagtccccctctggttccgatgtcagtctcagacacttagcgtgataaacccggggacagagctcacagcaaaggacttggccttcccggtgacaaacccagcagtagaaatcattccgtccatcctgcggtacaacatcaacagggtctgtggtgagtggctgcttcatatagtaaaacggaccatgtcttagttctgactgctccttattgttactgttcagtaagccaggtttctttttctttttaatggggcttgttgatgtgtcctgcggcgagtggccattggaagaatgtggagggctggggaactttcttttctgggctgttctctctgcagagccaggatctttggagcgagtagagatatccatgccctctaccacctcctgttctgtttttatttcctcttcagccaagctctgtggatgcattgttaacactgtgtaatgtcaatacttat

SEQ ID NO: 18763 - RNA, 4520 nt, Homo sapiens
  source 1..4520: mol_type = other RNA
tgagtgtgtgtgtgtgagtgtgtttaaaggaaccacaaagcaaagataaggtttctctttttttcagagttcatgatcctaagactttctgtgttctctcctgtgactgagctgagtggggcttgtttgtttctcttctgtaaacaaggatattgttttttcccttttaggagtagagtcatcatttcaatcacatgaaagaaactagcttctccctgtgtccgtctggtccggagagcttgcgttttaggaacgtggtaacgtagtagctgaaaggagccaacggcttgatgggatagtctgtgccgaaactcccgatcccaacatgctgcgtacagacacacgagcgaaaacggttcgccctcccctgggtatccaaggatgaggacgtgagtatgaaagtggtccccgggcccagtatccattccgtcgtgtgacagacaggctaactgaccatcccttctccaataccaaaacattcttttttgttgttggggttggttgcttttttttttttttttaaatcgtttttctttttctttttttttttttaataagttaaagttaatacaaatataaaaaggggaaagtcctctagattcaatgacatccacaaattgtacattatttacaccaaaagcacagggctcgtgtgggtgaacagtctgcagtcaaagccgatgctgggtgtcctgtagtgtagcagcccccgcgccgggggctcaggctcaactgagggttttgtcattttcaagtctgaaagtggctgttctcctgcctttgttgtttcttcttttcctggcgtctgggtttttctcccaatggggtgggtggtttgtgtcccgattcactgctagtcccagaaggtgtccagccgagactctttcgggaggaggctcttcgtgctggtactggtgttgtgatcggaacgtgtcgatcccctcttctcatcactgctgctccaactggatttattactccgggaatggtacttctgggcggggtagttggggtgcggctggtggtctgtggtggttggggcataggcaggttgcttgtcacaccttttgctaacagagccttggttggagcctaagagaatggaggagggcgtctctctggagccagaaaggtcaagggtcgagccactctccttgcttttctcagctgacgtctccttctctttggaggcgctggccgtttctgaaggtgctgattgtgtgctcgaggagctcccctgggaggacttatttagtgtttctgtgttcacctcagcatccgcttcctgctgaggagcagtagctgactgggtgcaggacttcatgtgctcaggccagtgggcttgctggcaggggtagtcacagtagctggtgttccaacagcagtaaaagatggcctccttcttgcagttggcgcaccactgcttcttcttggtctcatccaccgcctgctgcttctccaactccagctgcttcttcacctcggcgatgagccggtcccgctcctgctccaggctctgccgcatctccgccatggtcagctctaagttgtgtttcatttcggagagctcttgctggtgcagccactggagcttctctatctcgatcctcagcctgcgaatctcagctattgtgcttccagtagtgtttttagaaagatcgttgtatatttctgtcattgttccttttattgcatccatcattttgctagtgtacttggcaatatcagcggcgacatcagctgaggcagtggcgatgggcaggtcagcgttgactgaggacacaagggtgctcatggaccccgagctggtgaccaggggcgatgactgtgtgctggtcaccagggtgatggtggacgtggatgggctctgtgtgatctccttctgctggacagttgatgagttccacacgacccgctgcacggccggggcagtctccttcggtaaaagcggcctctgctttttcactgggcttcctgtggcggcgggggccggggccgtgacggtgaccgtggaggacgtgctggtggtggctgtggcgccagccgcggaagtttgggcggaagagcgggtgagcaccggtgtttccgggggagaatggctgcccaccgtcgtggatggtggagttttacctacaacatcctgtttgggagatggttctttgggttccttcttattttttcgaccctcccgcccagaatggtcttctcctaaatctatgacaagttcgctctctgaatcagagtccaggcccaaatggactgttggggaatccgtctcatcttttcccttcagtttatcctttatggggtgaggtgaaggttttgccttttcggaaaagtccttctcaggctcagggctggccttgtccttgactgctccagggtctgccttctcgctggctggtgacgtgcttttcagctcctctttaatctccactgggtttgtaggcttgggcttttttttaacagcagatggctctttgtccatctgacaaccttctttgtcctctgtgtcttctggctcgttcttagacttctgctcatcatcactgatatactcactatcgctactatctgacttctcagaatcctccgaatcgctgtgctctacggccgtatagacatcttccgagatttcatttatgcctaattgtgctttgcaactctctatggtcttgtcaagattcagctggaacctgctacgaatctggcgcttgggagagatgagaggaacaggggtggactgttgctggaccgactcgctcagctccttcaaatccatctcagctttgcttcgatccaggttaagattcaggatgctgccggtggtggaggttttgtccgttttcgtcgtgataggagctgacagttgaggagagaagggctttgggctgccggataaactccctgcttgtcccgtcttggtggaggctggtgaagctgtgctcttatccaggaagtccatggactcctcgctcgcactgaagtggctcgacgtggccttcttctcagcatcctgctccacgtcggagcccgtgtgcacagaagagtttgtgctcatgggggagcgcggcatatccgacaaggaaatccggcggcctgtgcccccactcagcacaggcttgctcatcaggatcttgggggatgccgtcatgtcaaagttgagcttgaccttctcctgcttgtctatcttggcagtgccggcgctggggttggtgggatcgagcagcatttgatactggctgttgggtgtgtagggtgtcctaaatggagagtaattaaaaaccccaaacttcctgcggatgttctccacgtaaacctccatctcttgcatggcactgttgaagatgctcttagtctttttcacagaaaaaggaatttctttagacatgaggtagcaattatttattggaacccaggccctgtcatgttgtccaaagaatcgggcatcgacctgcccgtctttatcccttagagcttttgcaggccagaatggaaaccccttcagtttggcccagaccaaaggatgtggattgctacaaggctcacaaaaccagttatctcgtttttggcaagcagctagataacattctggacatacttcgatttcattcatctcatgttcacagattttgatgactactttcgctatttgcgtcaatttgtgatttcccccattataaatgatgcagttgtgcaaaatccactttgcatcagccaggaaggcttctgtgcagccatacattttctttttcgcattcttttccaatgtacaaaggtccattggatggaagatgtattccgcatagtcagggtgctgttccaatggaacgggcttctggaatgcatctgtccctggctgtttcattttctgaatggcaaacttgagcaggtaggataactgttcaatggtgagcattgtcatggctttactctgggtctcgatgcattctgctactgtaattttctcacattcaggacaaaaccagtccccctctggttccgatgtcagtctcagacacttagcgtgataaacccggggacagagctcacagcaaaggacttggccttcccggtgacaaacccagcagtagaaatcattccgtccatcctgcggtacaacatcaacagggtctgtggtgagtggctgcttcatatagtaaaacggaccatgtcttagttctgactgctccttattgttactgttcagtaagccaggtttctttttctttttaatggggcttgttgatgtgtcctgcggcgagtggccattggaagaatgtggagggctggggaactttcttttctgggctgttctctctgcagagccaggatctttggagcgagtagagatatccatgccctctaccacctcctgttctgtttttatttcctcttcagccaagccaacaaatgttcaagcaaccgtctcatttttccacagttaggaagagagaacaggctggcagatttgggactctgtggatgcattgttaacactgtgtaatgtcaatacttat

SEQ ID NO: 18764 - RNA, 4449 nt, Homo sapiens
  source 1..4449: mol_type = other RNA
tgagtgtgtgtgtgtgagtgtgtttaaaggaaccacaaagcaaagataaggtttctctttttttcagagttcatgatcctaagactttctgtgttctctcctgtgactgagctgagtggggcttgtttgtttctcttctgtaaacaaggatattgttttttcccttttaggagtagagtcatcatttcaatcacatgaaagaaactagcttctccctgtgtccgtctggtccggagagcttgcgttttaggaacgtggtaacgtagtagctgaaaggagccaacggcttgatgggatagtctgtgccgaaactcccgatcccaacatgctgcgtacagacacacgagcgaaaacggttcgccctcccctgggtatccaaggatgaggacgtgagtatgaaagtggtccccgggcccagtatccattccgtcgtgtgacagacaggctaactgaccatcccttctccaataccaaaacattcttttttgttgttggggttggttgcttttttttttttttttaaatcgtttttctttttctttttttttttttaataagttaaagttaatacaaatataaaaaggggaaagtcctctagattcaatgacatccacaaattgtacattatttacaccaaaagcacagggctcgtgtgggtgaacagtctgcagtcaaagccgatgctgggtgtcctgtagtgtagcagcccccgcgccgggggctcaggctcaactgagggttttgtcattttcaagtctgaaagtggctgttctcctgcctttgttgtttcttcttttcctggcgtctgggtttttctcccaatggggtgggtggtttgtgtcccgattcactgctagtcccagaaggtgtccagccgagactctttcgggaggaggctcttcgtgctggtactggtgttgtgatcggaacgtgtcgatcccctcttctcatcactgctgctccaactggatttattactccgggaatggtacttctgggcggggtagttggggtgcggctggtggtctgtggtggttggggcataggcaggttgcttgtcacaccttttgctaacagagccttggttggagcctaagagaatggaggagggcgtctctctggagccagaaaggtcaagggtcgagccactctccttgcttttctcagctgacgtctccttctctttggaggcgctggccgtttctgaaggtgctgattgtgtgctcgaggagctcccctgggaggacttatttagtgtttctgtgttcacctcagcatccgcttcctgctgaggagcagtagctgactgggtgcaggacttcatgtgctcaggccagtgggcttgctggcaggggtagtcacagtagctggtgttccaacagcagtaaaagatggcctccttcttgcagttggcgcaccactgcttcttcttggtctcatccaccgcctgctgcttctccaactccagctgcttcttcacctcggcgatgagccggtcccgctcctgctccaggctctgccgcatctccgccatggtcagctctaagttgtgtttcatttcggagagctcttgctggtgcagccactggagcttctctatctcgatcctcagcctgcgaatctcagctattgtgcttccagtagtgtttttagaaagatcgttgtatatttctgtcattgttccttttattgcatccatcattttgctagtgtacttggcaatatcagcggcgacatcagctgaggcagtggcgatgggcaggtcagcgttgactgaggacacaagggtgctcatggaccccgagctggtgaccaggggcgatgactgtgtgctggtcaccagggtgatggtggacgtggatgggctctgtgtgatctccttctgctggacagttgatgagttccacacgacccgctgcacggccggggcagtctccttcggtaaaagcggcctctgctttttcactgggcttcctgtggcggcgggggccggggccgtgacggtgaccgtggaggacgtgctggtggtggctgtggcgccagccgcggaagtttgggcggaagagcgggtgagcaccggtgtttccgggggagaatggctgcccaccgtcgtggatggtggagttttacctacaacatcctgtttgggagatggttctttgggttccttcttattttttcgaccctcccgcccagaatggtcttctcctaaatctatgacaagttcgctctctgaatcagagtccaggcccaaatggactgttggggaatccgtctcatcttttcccttcagtttatcctttatggggtgaggtgaaggttttgccttttcggaaaagtccttctcaggctcagggctggccttgtccttgactgctccagggtctgccttctcgctggctggtgacgtgcttttcagctcctctttaatctccactgggtttgtaggcttgggcttttttttaacagcagatggctctttgtccatctgacaaccttctttgtcctctgtgtcttctggctcgttcttagacttctgctcatcatcactgatatactcactatcgctactatctgacttctcagaatcctccgaatcgctgtgctctacggccgtatagacatcttccgagatttcatttatgcctaattgtgctttgcaactctctatggtcttgtcaagattcagctggaacctgctacgaatctggcgcttgggagagatgagaggaacaggggtggactgttgctggaccgactcgctcagctccttcaaatccatctcagctttgcttcgatccaggttaagattcaggatgctgccggtggtggaggttttgtccgttttcgtcgtgataggagctgacagttgaggagagaagggctttgggctgccggataaactccctgcttgtcccgtcttggtggaggctggtgaagctgtgctcttatccaggaagtccatggactcctcgctcgcactgaagtggctcgacgtggccttcttctcagcatcctgctccacgtcggagcccgtgtgcacagaagagtttgtgctcatgggggagcgcggcatatccgacaaggaaatccggcggcctgtgcccccactcagcacaggcttgctcatcaggatcttgggggatgccgtcatgtcaaagttgagcttgaccttctcctgcttgtctatcttggcagtgccggcgctggggttggtgggatcgagcagcatttgatactggctgttgggtgtgtagggtgtcctaaatggagagtaattaaaaaccccaaacttcctgcggatgttctccacgtaaacctccatctcttgcatggcactgttgaagatgctcttagtctttttcacagaaaaaggaatttctttagacatgaggtagcaattatttattggaacccaggccctgtcatgttgtccaaagaatcgggcatcgacctgcccgtctttatcccttagagcttttgcaggccagaatggaaaccccttcagtttggcccagaccaaaggatgtggattgctacaaggctcacaaaaccagttatctcgtttttggcaagcagctagataacattctggacatacttcgatttcattcatctcatgttcacagattttgatgactactttcgctatttgcgtcaatttgtgatttcccccattataaatgatgcagttgtgcaaaatccactttgcatcagccaggaaggcttctgtgcagccatacattttctttttcgcattcttttccaatgtacaaaggtccattggatggaagatgtattccgcatagtcagggtgctgttccaatggaacgggcttctggaatgcatctgtccctggctgtttcattttctgaatggcaaacttgagcaggtaggataactgttcaatggtgagcattgtcatggctttactctgggtctcgatgcattctgctactgtaattttctcacattcaggacaaaaccagtccccctctggttccgatgtcagtctcagacacttagcgtgataaacccggggacagagctcacagcaaaggacttggccttcccggtgacaaacccagcagtagaaatcattccgtccatcctgcggtacaacatcaacagggtctgtggtgagtggctgcttcatatagtaaaacggaccatgtcttagttctgactgctccttattgttactgttcagtaagccaggtttctttttctttttaatggggcttgttgatgtgtcctgcggcgagtggccattggaagaatgtggagggctggggaactttcttttctgggctgttctctctgcagagccaggatctttggagcgagtagagatatccatgccctctaccacctcctgttctgtttttatttcctcttcagccaagctctgtggatgcattgttaacactgtgtaatgtcaatacttat

SEQ ID NO: 18765 - RNA, 4374 nt, Homo sapiens
  source 1..4374: mol_type = other RNA
tgagtgtgtgtgtgtgagtgtgtttaaaggaaccacaaagcaaagataaggtttctctttttttcagagttcatgatcctaagactttctgtgttctctcctgtgactgagctgagtggggcttgtttgtttctcttctgtaaacaaggatattgttttttcccttttaggagtagagtcatcatttcaatcacatgaaagaaactagcttctccctgtgtccgtctggtccggagagcttgcgttttaggaacgtggtaacgtagtagctgaaaggagccaacggcttgatgggatagtctgtgccgaaactcccgatcccaacatgctgcgtacagacacacgagcgaaaacggttcgccctcccctgggtatccaaggatgaggacgtgagtatgaaagtggtccccgggcccagtatccattccgtcgtgtgacagacaggctaactgaccatcccttctccaataccaaaacattcttttttgttgttggggttggttgcttttttttttttttttaaatcgtttttctttttctttttttttttttaataagttaaagttaatacaaatataaaaaggggaaagtcctctagattcaatgacatccacaaattgtacattatttacaccaaaagcacagggctcgtgtgggtgaacagtctgcagtcaaagccgatgctgggtgtcctgtagtgtagcagcccccgcgccgggggctcaggctcaactgagggttttgtcattttcaagtctgaaagtggctgttctcctgcctttgttgtttcttcttttcctggcgtctgggtttttctcccaatggggtgggtggtttgtgtcccgattcactgctagtcccagaaggtgtccagccgagactctttcgggaggaggctcttcgtgctggtactggtgttgtgatcggaacgtgtcgatcccctcttctcatcactgctgctccaactggatttattactccgggaatggtacttctgggcggggtagttggggtgcggctggtggtctgtggtggttggggcataggcaggttgcttgtcacaccttttgctaacagagccttggttggagcctaagagaatggaggagggcgtctctctggagccagaaaggtcaagggtcgagccactctccttgcttttctcagctgacgtctccttctctttggaggcgctggccgtttctgaaggtgctgattgtgtgctcgaggagctcccctgggaggacttatttagtgtttctgtgttcacctcagcatccgcttcctgctgaggagcagtagctgactgggtgcaggacttcatgtgctcaggccagtgggcttgctggcaggggtagtcacagtagctggtgttccaacagcagtaaaagatggcctccttcttgcagttggcgcaccactgcttcttcttggtctcatccaccgcctgctgcttctccaactccagctgcttcttcacctcggcgatgagccggtcccgctcctgctccaggctctgccgcatctccgccatggtcagctctaagttgtgtttcatttcggagagctcttgctggtgcagccactggagcttctctatctcgatcctcagcctgcgaatctcagctattgtgcttccagtagtgtttttagaaagatcgttgtatatttctgtcattgttccttttattgcatccatcattttgctagtgtacttggcaatatcagcggcgacatcagctgaggcagtggcgatgggcaggtcagcgttgactgaggacacaagggtgctcatggaccccgagctggtgaccaggggcgatgactgtgtgctggtcaccagggtgatggtggacgtggatgggctctgtgtgatctccttctgctggacagttgatgagttccacacgacccgctgcacggccggggcagtctccttcggtaaaagcggcctctgctttttcactgggcttcctgtggcggcgggggccggggccgtgacggtgaccgtggaggacgtgctggtggtggctgtggcgccagccgcggaagtttgggcggaagagcgggtgagcaccggtgtttccgggggagaatggctgcccaccgtcgtggatggtggagttttacctacaacatcctgtttgggagatggttctttgggttccttcttattttttcgaccctcccgcccagaatggtcttctcctaaatctatgacaagttcgctctctgaatcagagtccaggcccaaatggactgttggggaatccgtctcatcttttcccttcagtttatcctttatggggtgaggtgaaggttttgccttttcggaaaagtccttctcaggctcagggctggccttgtccttgactgctccagggtctgccttctcgctggctggtgacgtgcttttcagctcctctttaatctccactgggtttgtaggcttgggcttttttttaacagcagatggctctttgtccatctgacaaccttctttgtcctctgtgtcttctggctcgttcttagacttctgctcatcatcactgatatactcactatcgctactatctgacttctcagaatcctccgaatcgctgtgctctacggccgtatagacatcttccgagatttcatttatgcctaattgtgctttgcaactctctatggtcttgtcaagattcagctggaacctgctacgaatctggcgcttgggagagatgagaggaacaggggtggactgttgctggaccgactcgctcagctccttcaaatccatctcagctttgcttcgatccaggttaagattcaggatgctgccggtggtggaggttttgtccgttttcgtcgtgataggagctgacagttgaggagagaagggctttgggctgccggataaactccctgcttgtcccgtcttggtggaggctggtgaagctgtgctcttatccaggaagtccatggactcctcgctcgcactgaagtggctcgacgtggccttcttctcagcatcctgctccacgtcggagcccgtgtgcacagaagagtttgtgctcatgggggagcgcggcatatccgacaaggaaatccggcggcctgtgcccccactcagcacaggcttgctcatcaggatcttgggggatgccgtcatgtcaaagttgagcttgaccttctcctgcttgtctatcttggcagtgccggcgctggggttggtgggatcgagcagcatttgatactggctgttgggtgtgtagggtgtcctaaatggagagtaattaaaaaccccaaacttcctgcggatgttctccacgtaaacctccatctcttgcatggcactgttgaagatgctcttagtctttttcacagaaaaaggaatttctttagacatgaggtagcaattatttattggaacccaggccctgtcatgttgtccaaagaatcgggcatcgacctgcccgtctttatcccttagagcttttgcaggccagaatggaaaccccttcagtttggcccagaccaaaggatgtggattgctacaaggctcacaaaaccagttatctcgtttttggcaagcagctagataacattctggacatacttcgatttcattcatctcatgttcacagattttgatgactactttcgctatttgcgtcaatttgtgatttcccccattataaatgatgcagttgtgcaaaatccactttgcatcagccaggaaggcttctgtgcagccatacattttctttttcgcattcttttccaatgtacaaaggtccattggatggaagatgtattccgcatagtcagggtgctgttccaatggaacgggcttctggaatgcatctgtccctggctgtttcattttctgaatggcaaacttgagcaggtaggataactgttcaatggtgagcattgtcatggctttactctgggtctcgatgcattctgctactgtaattttctcacattcaggacaaaaccagtccccctctggttccgatgtcagtctcagacacttagcgtgataaacccggggacagagctcacagcaaaggacttggccttcccggtgacaaacccagcagtagaaatcattccgtccatcctgctccttattgttactgttcagtaagccaggtttctttttctttttaatggggcttgttgatgtgtcctgcggcgagtggccattggaagaatgtggagggctggggaactttcttttctgggctgttctctctgcagagccaggatctttggagcgagtagagatatccatgccctctaccacctcctgttctgtttttatttcctcttcagccaagctctgtggatgcattgttaacactgtgtaatgtcaatacttat

SEQ ID NO: 18766 - RNA, 4580 nt, Homo sapiens
  source 1..4580: mol_type = other RNA
tgagtgtgtgtgtgtgagtgtgtttaaaggaaccacaaagcaaagataaggtttctctttttttcagagttcatgatcctaagactttctgtgttctctcctgtgactgagctgagtggggcttgtttgtttctcttctgtaaacaaggatattgttttttcccttttaggagtagagtcatcatttcaatcacatgaaagaaactagcttctccctgtgtccgtctggtccggagagcttgcgttttaggaacgtggtaacgtagtagctgaaaggagccaacggcttgatgggatagtctgtgccgaaactcccgatcccaacatgctgcgtacagacacacgagcgaaaacggttcgccctcccctgggtatccaaggatgaggacgtgagtatgaaagtggtccccgggcccagtatccattccgtcgtgtgacagacaggctaactgaccatcccttctccaataccaaaacattcttttttgttgttggggttggttgcttttttttttttttttaaatcgtttttctttttctttttttttttttaataagttaaagttaatacaaatataaaaaggggaaagtcctctagattcaatgacatccacaaattgtacattatttacaccaaaagcacagggctcgtgtgggtgaacagtctgcagtcaaagccgatgctgggtgtcctgtagtgtagcagcccccgcgccgggggctcaggctcaactgagggttttgtcattttcaagtctgaaagtggctgttctcctgcctttgttgtttcttcttttcctggcgtctgggtttttctcccaatggggtgggtggtttgtgtcccgattcactgctagtcccagaaggtgtccagccgagactctttcgggaggaggctcttcgtgctggtactggtgttgtgatcggaacgtgtcgatcccctcttctcatcactgctgctccaactggatttattactccgggaatggtacttctgggcggggtagttggggtgcggctggtggtctgtggtggttggggcataggcaggttgcttgtcacaccttttgctaacagagccttggttggagcctaagagaatggaggagggcgtctctctggagccagaaaggtcaagggtcgagccactctccttgcttttctcagctgacgtctccttctctttggaggcgctggccgtttctgaaggtgctgattgtgtgctcgaggagctcccctgggaggacttatttagtgtttctgtgttcacctcagcatccgcttcctgctgaggagcagtagctgactgggtgcaggacttcatgtgctcaggccagtgggcttgctggcaggggtagtcacagtagctggtgttccaacagcagtaaaagatggcctccttcttgcagttggcgcaccactgcttcttcttggtctcatccaccgcctgctgcttctccaactccagctgcttcttcacctcggcgatgagccggtcccgctcctgctccaggctctgccgcatctccgccatggtcagctctaagttgtgtttcatttcggagagctcttgctggtgcagccactggagcttctctatctcgatcctcagcctgcgaatctcagctattgtgcttccagtagtgtttttagaaagatcgttgtatatttctgtcattgttccttttattgcatccatcattttgctagtgtacttggcaatatcagcggcgacatcagctgaggcagtggcgatgggcaggtcagcgttgactgaggacacaagggtgctcatggaccccgagctggtgaccaggggcgatgactgtgtgctggtcaccagggtgatggtggacgtggatgggctctgtgtgatctccttctgctggacagttgatgagttccacacgacccgctgcacggccggggcagtctccttcggtaaaagcggcctctgctttttcactgggcttcctgtggcggcgggggccggggccgtgacggtgaccgtggaggacgtgctggtggtggctgtggcgccagccgcggaagtttgggcggaagagcgggtgagcaccggtgtttccgggggagaatggctgcccaccgtcgtggatggtggagttttacctacaacatcctgtttgggagatggttctttgggttccttcttattttttcgaccctcccgcccagaatggtcttctcctaaatctatgacaagttcgctctctgaatcagagtccaggcccaaatggactgttggggaatccgtctcatcttttcccttcagtttatcctttatggggtgaggtgaaggttttgccttttcggaaaagtccttctcaggctcagggctggccttgtccttgactgctccagggtctgccttctcgctggctggtgacgtgcttttcagctcctctttaatctccactgggtttgtaggcttgggcttttttttaacagcagatggctctttgtccatctgacaaccttctttgtcctctgtgtcttctggctcgttcttagacttctgctcatcatcactgatatactcactatcgctactatctgacttctcagaatcctccgaatcgctgtgctctacggccgtatagacatcttccgagatttcatttatgcctaattgtgctttgcaactctctatggtcttgtcaagattcagctggaacctgctacgaatctggcgcttgggagagatgagaggaacaggggtggactgttgctggaccgactcgctcagctccttcaaatccatctcagctttgcttcgatccaggttaagattcaggatgctgccggtggtggaggttttgtccgttttcgtcgtgataggagctgacagttgaggagagaagggctttgggctgccggataaactccctgcttgtcccgtcttggtggaggctggtgaagctgtgctcttatccaggaagtccatggactcctcgctcgcactgaagtggctcgacgtggccttcttctcagcatcctgctccacgtcggagcccgtgtgcacagaagagtttgtgctcatgggggagcgcggcatatccgacaaggaaatccggcggcctgtgcccccactcagcacaggcttgctcatcaggatcttgggggatgccgtcatgtcaaagttgagcttgaccttctcctgcttgtctatcttggcagtgccggcgctggggttggtgggatcgagcagcatttgatactggctgttgggtgtgtagggtgtcctaaatggagagtaattaaaaaccccaaacttcctgcggatgttctccacgtaaacctccatctcttgcatggcactgttgaagatgctcttagtctttttcacagaaaaaggaatttctttagacatgaggtagcaattatttattggaacccaggccctgtcatgttgtccaaagaatcgggcatcgacctgcccgtctttatcccttagagcttttgcaggccagaatggaaaccccttcagtttggcccagaccaaaggatgtggattgctacaaggctcacaaaaccagttatctcgtttttggcaagcagctagataacattctggacatacttcgatttcattcatcttgttacttaagatgctgataaaactgggtactatttaatgacaagaggagtaattaaatgaatgtccatgtgttgtatgtaatactatacagccatgaaaaattctgttcttcctacgagtttaattacctcatgttcacagattttgatgactactttcgctatttgcgtcaatttgtgatttcccccattataaatgatgcagttgtgcaaaatccactttgcatcagccaggaaggcttctgtgcagccatacattttctttttcgcattcttttccaatgtacaaaggtccattggatggaagatgtattccgcatagtcagggtgctgttccaatggaacgggcttctggaatgcatctgtccctggctgtttcattttctgaatggcaaacttgagcaggtaggataactgttcaatggtgagcattgtcatggctttactctgggtctcgatgcattctgctactgtaattttctcacattcaggacaaaaccagtccccctctggttccgatgtcagtctcagacacttagcgtgataaacccggggacagagctcacagcaaaggacttggccttcccggtgacaaacccagcagtagaaatcattccgtccatcctgcggtacaacatcaacagggtctgtggtgagtggctgcttcatatagtaaaacggaccatgtcttagttctgactgctccttattgttactgttcagtaagccaggtttctttttctttttaatggggcttgttgatgtgtcctgcggcgagtggccattggaagaatgtggagggctggggaactttcttttctgggctgttctctctgcagagccaggatctttggagcgagtagagatatccatgccctctaccacctcctgttctgtttttatttcctcttcagccaagctctgtggatgcattgttaacactgtgtaatgtcaatacttat

SEQ ID NO: 18767 - RNA, 4293 nt, Homo sapiens
  source 1..4293: mol_type = other RNA
tgagtgtgtgtgtgtgagtgtgtttaaaggaaccacaaagcaaagataaggtttctctttttttcagagttcatgatcctaagactttctgtgttctctcctgtgactgagctgagtggggcttgtttgtttctcttctgtaaacaaggatattgttttttcccttttaggagtagagtcatcatttcaatcacatgaaagaaactagcttctccctgtgtccgtctggtccggagagcttgcgttttaggaacgtggtaacgtagtagctgaaaggagccaacggcttgatgggatagtctgtgccgaaactcccgatcccaacatgctgcgtacagacacacgagcgaaaacggttcgccctcccctgggtatccaaggatgaggacgtgagtatgaaagtggtccccgggcccagtatccattccgtcgtgtgacagacaggctaactgaccatcccttctccaataccaaaacattcttttttgttgttggggttggttgcttttttttttttttttaaatcgtttttctttttctttttttttttttaataagttaaagttaatacaaatataaaaaggggaaagtcctctagattcaatgacatccacaaattgtacattatttacaccaaaagcacagggctcgtgtgggtgaacagtctgcagtcaaagccgatgctgggtgtcctgtagtgtagcagcccccgcgccgggggctcaggctcaactgagggttttgtcattttcaagtctgaaagtggctgttctcctgcctttgttgtttcttcttttcctggcgtctgggtttttctcccaatggggtgggtggtttgtgtcccgattcactgctagtcccagaaggtgtccagccgagactctttcgggaggaggctcttcgtgctggtactggtgttgtgatcggaacgtgtcgatcccctcttctcatcactgctgctccaactggatttattactccgggaatggtacttctgggcggggtagttggggtgcggctggtggtctgtggtggttggggcataggcaggttgcttgtcacaccttttgctaacagagccttggttggagcctaagagaatggaggagggcgtctctctggagccagaaaggtcaagggtcgagccactctccttgcttttctcagctgacgtctccttctctttggaggcgctggccgtttctgaaggtgctgattgtgtgctcgaggagctcccctgggaggacttatttagtgtttctgtgttcacctcagcatccgcttcctgctgaggagcagtagctgactgggtgcaggacttcatgtgctcaggccagtgggcttgctggcaggggtagtcacagtagctggtgttccaacagcagtaaaagatggcctccttcttgcagttggcgcaccactgcttcttcttggtctcatccaccgcctgctgcttctccaactccagctgcttcttcacctcggcgatgagccggtcccgctcctgctccaggctctgccgcatctccgccatggtcagctctaagttgtgtttcatttcggagagctcttgctggtgcagccactggagcttctctatctcgatcctcagcctgcgaattttgctagtgtacttggcaatatcagcggcgacatcagctgaggcagtggcgatgggcaggtcagcgttgactgaggacacaagggtgctcatggaccccgagctggtgaccaggggcgatgactgtgtgctggtcaccagggtgatggtggacgtggatgggctctgtgtgatctccttctgctggacagttgatgagttccacacgacccgctgcacggccggggcagtctccttcggtaaaagcggcctctgctttttcactgggcttcctgtggcggcgggggccggggccgtgacggtgaccgtggaggacgtgctggtggtggctgtggcgccagccgcggaagtttgggcggaagagcgggtgagcaccggtgtttccgggggagaatggctgcccaccgtcgtggatggtggagttttacctacaacatcctgtttgggagatggttctttgggttccttcttattttttcgaccctcccgcccagaatggtcttctcctaaatctatgacaagttcgctctctgaatcagagtccaggcccaaatggactgttggggaatccgtctcatcttttcccttcagtttatcctttatggggtgaggtgaaggttttgccttttcggaaaagtccttctcaggctcagggctggccttgtccttgactgctccagggtctgccttctcgctggctggtgacgtgcttttcagctcctctttaatctccactgggtttgtaggcttgggcttttttttaacagcagatggctctttgtccatctgacaaccttctttgtcctctgtgtcttctggctcgttcttagacttctgctcatcatcactgatatactcactatcgctactatctgacttctcagaatcctccgaatcgctgtgctctacggccgtatagacatcttccgagatttcatttatgcctaattgtgctttgcaactctctatggtcttgtcaagattcagctggaacctgctacgaatctggcgcttgggagagatgagaggaacaggggtggactgttgctggaccgactcgctcagctccttcaaatccatctcagctttgcttcgatccaggttaagattcaggatgctgccggtggtggaggttttgtccgttttcgtcgtgataggagctgacagttgaggagagaagggctttgggctgccggataaactccctgcttgtcccgtcttggtggaggctggtgaagctgtgctcttatccaggaagtccatggactcctcgctcgcactgaagtggctcgacgtggccttcttctcagcatcctgctccacgtcggagcccgtgtgcacagaagagtttgtgctcatgggggagcgcggcatatccgacaaggaaatccggcggcctgtgcccccactcagcacaggcttgctcatcaggatcttgggggatgccgtcatgtcaaagttgagcttgaccttctcctgcttgtctatcttggcagtgccggcgctggggttggtgggatcgagcagcatttgatactggctgttgggtgtgtagggtgtcctaaatggagagtaattaaaaaccccaaacttcctgcggatgttctccacgtaaacctccatctcttgcatggcactgttgaagatgctcttagtctttttcacagaaaaaggaatttctttagacatgaggtagcaattatttattggaacccaggccctgtcatgttgtccaaagaatcgggcatcgacctgcccgtctttatcccttagagcttttgcaggccagaatggaaaccccttcagtttggcccagaccaaaggatgtggattgctacaaggctcacaaaaccagttatctcgtttttggcaagcagctagataacattctggacatacttcgatttcattcatctcatgttcacagattttgatgactactttcgctatttgcgtcaatttgtgatttcccccattataaatgatgcagttgtgcaaaatccactttgcatcagccaggaaggcttctgtgcagccatacattttctttttcgcattcttttccaatgtacaaaggtccattggatggaagatgtattccgcatagtcagggtgctgttccaatggaacgggcttctggaatgcatctgtccctggctgtttcattttctgaatggcaaacttgagcaggtaggataactgttcaatggtgagcattgtcatggctttactctgggtctcgatgcattctgctactgtaattttctcacattcaggacaaaaccagtccccctctggttccgatgtcagtctcagacacttagcgtgataaacccggggacagagctcacagcaaaggacttggccttcccggtgacaaacccagcagtagaaatcattccgtccatcctgctccttattgttactgttcagtaagccaggtttctttttctttttaatggggcttgttgatgtgtcctgcggcgagtggccattggaagaatgtggagggctggggaactttcttttctgggctgttctctctgcagagccaggatctttggagcgagtagagatatccatgccctctaccacctcctgttctgtttttatttcctcttcagccaagctctgtggatgcattgttaacactgtgtaatgtcaatacttat

SEQ ID NO: 18768 - RNA, 4047 nt, Homo sapiens
  source 1..4047: mol_type = other RNA
tgagtgtgtgtgtgtgagtgtgtttaaaggaaccacaaagcaaagataaggtttctctttttttcagagttcatgatcctaagactttctgtgttctctcctgtgactgagctgagtggggcttgtttgtttctcttctgtaaacaaggatattgttttttcccttttaggagtagagtcatcatttcaatcacatgaaagaaactagcttctccctgtgtccgtctggtccggagagcttgcgttttaggaacgtggtaacgtagtagctgaaaggagccaacggcttgatgggatagtctgtgccgaaactcccgatcccaacatgctgcgtacagacacacgagcgaaaacggttcgccctcccctgggtatccaaggatgaggacgtgagtatgaaagtggtccccgggcccagtatccattccgtcgtgtgacagacaggctaactgaccatcccttctccaataccaaaacattcttttttgttgttggggttggttgcttttttttttttttttaaatcgtttttctttttctttttttttttttaataagttaaagttaatacaaatataaaaaggggaaagtcctctagattcaatgacatccacaaattgtacattatttacaccaaaagcacagggctcgtgtgggtgaacagtctgcagtcaaagccgatgctgggtgtcctgtagtgtagcagcccccgcgccgggggctcaggctcaactgagggttttgtcattttcaagtctgaaagtggctgttctcctgcctttgttgtttcttcttttcctggcgtctgggtttttctcccaatggggtgggtggtttgtgtcccgattcactgctagtcccagaaggtgtccagccgagactctttcgggaggaggctcttcgtgctggtactggtgttgtgatcggaacgtgtcgatcccctcttctcatcactgctgctccaactggatttattactccgggaatggtcagagccttggttggagcctaagagaatggaggagggcgtctctctggagccagaaaggtcaagggtcgagccactctccttgcttttctcagctgacgtctccttctctttggaggcgctggccgtttctgaaggtgctgattgtgtgctcgaggagctcccctgggaggacttatttagtgtttctgtgttcacctcagcatccgcttcctgctgaggagcagtagctgactgggtgcaggacttcatgtgctcaggccagtgggcttgctggcaggggtagtcacagtagctggtgttccaacagcagtaaaagatggcctccttcttgcagttggcgcaccactgcttcttcttggtctcatccaccgcctgctgcttctccaactccagctgcttcttcacctcggcgatgagccggtcccgctcctgctccaggctctgccgcatctccgccatggtcagctctaagttgtgtttcatttcggagagctcttgctggtgcagccactggagcttctctatctcgatcctcagcctgcgaatctcagctattgtgcttccagtagtgtttttagaaagatcgttgtatatttctgtcattgttccttttattgcatccatcattttgctagtgtacttggcaatatcagcggcgacatcagctgaggcagtggcgatgggcaggtcagcgttgactgaggacacaagggtgctcatggaccccgagctggtgaccaggggcgatgactgtgtgctggtcaccagggtgatggtggacgtggatgggctctgtgtgatctccttctgctggacagcatcctgtttgggagatggttctttgggttccttcttattttttcgaccctcccgcccagaatggtcttctcctaaatctatgacaagttcgctctctgaatcagagtccaggcccaaatggactgttggggaatccgtctcatcttttcccttcagtttatcctttatggggtgaggtgaaggttttgccttttcggaaaagtccttctcaggctcagggctggccttgtccttgactgctccagggtctgccttctcgctggctggtgacgtgcttttcagctcctctttaatctccactgggtttgtaggcttgggcttttttttaacagcagatggctctttgtccatctgacaaccttctttgtcctctgtgtcttctggctcgttcttagacttctgctcatcatcactgatatactcactatcgctactatctgacttctcagaatcctccgaatcgctgtgctctacggccgtatagacatcttccgagatttcatttatgcctaattgtgctttgcaactctctatggtcttgtcaagattcagctggaacctgctacgaatctggcgcttgggagagatgagaggaacaggggtggactgttgctggaccgactcgctcagctccttcaaatccatctcagctttgcttcgatccaggttaagattcaggatgctgccggtggtggaggttttgtccgttttcgtcgtgataggagctgacagttgaggagagaagggctttgggctgccggataaactccctgcttgtcccgtcttggtggaggctggtgaagctgtgctcttatccaggaagtccatggactcctcgctcgcactgaagtggctcgacgtggccttcttctcagcatcctgctccacgtcggagcccgtgtgcacagaagagtttgtgctcatgggggagcgcggcatatccgacaaggaaatccggcggcctgtgcccccactcagcacaggcttgctcatcaggatcttgggggatgccgtcatgtcaaagttgagcttgaccttctcctgcttgtctatcttggcagtgccggcgctggggttggtgggatcgagcagcatttgatactggctgttgggtgtgtagggtgtcctaaatggagagtaattaaaaaccccaaacttcctgcggatgttctccacgtaaacctccatctcttgcatggcactgttgaagatgctcttagtctttttcacagaaaaaggaatttctttagacatgaggtagcaattatttattggaacccaggccctgtcatgttgtccaaagaatcgggcatcgacctgcccgtctttatcccttagagcttttgcaggccagaatggaaaccccttcagtttggcccagaccaaaggatgtggattgctacaaggctcacaaaaccagttatctcgtttttggcaagcagctagataacattctggacatacttcgatttcattcatctcatgttcacagattttgatgactactttcgctatttgcgtcaatttgtgatttcccccattataaatgatgcagttgtgcaaaatccactttgcatcagccaggaaggcttctgtgcagccatacattttctttttcgcattcttttccaatgtacaaaggtccattggatggaagatgtattccgcatagtcagggtgctgttccaatggaacgggcttctggaatgcatctgtccctggctgtttcattttctgaatggcaaacttgagcaggtaggataactgttcaatggtgagcattgtcatggctttactctgggtctcgatgcattctgctactgtaattttctcacattcaggacaaaaccagtccccctctggttccgatgtcagtctcagacacttagcgtgataaacccggggacagagctcacagcaaaggacttggccttcccggtgacaaacccagcagtagaaatcattccgtccatcctgctccttattgttactgttcagtaagccaggtttctttttctttttaatggggcttgttgatgtgtcctgcggcgagtggccattggaagaatgtggagggctggggaactttcttttctgggctgttctctctgcagagccaggatctttggagcgagtagagatatccatgccctctaccacctcctgttctgtttttatttcctcttcagccaagctctgtggatgcattgttaacactgtgtaatgtcaatacttat

SEQ ID NO: 18769 - RNA, 4585 nt, Homo sapiens
  source 1..4585: mol_type = other RNA
tgagtgtgtgtgtgtgagtgtgtttaaaggaaccacaaagcaaagataaggtttctctttttttcagagttcatgatcctaagactttctgtgttctctcctgtgactgagctgagtggggcttgtttgtttctcttctgtaaacaaggatattgttttttcccttttaggagtagagtcatcatttcaatcacatgaaagaaactagcttctccctgtgtccgtctggtccggagagcttgcgttttaggaacgtggtaacgtagtagctgaaaggagccaacggcttgatgggatagtctgtgccgaaactcccgatcccaacatgctgcgtacagacacacgagcgaaaacggttcgccctcccctgggtatccaaggatgaggacgtgagtatgaaagtggtccccgggcccagtatccattccgtcgtgtgacagacaggctaactgaccatcccttctccaataccaaaacattcttttttgttgttggggttggttgcttttttttttttttttaaatcgtttttctttttctttttttttttttaataagttaaagttaatacaaatataaaaaggggaaagtcctctagattcaatgacatccacaaattgtacattatttacaccaaaagcacagggctcgtgtgggtgaacagtctgcagtcaaagccgatgctgggtgtcctgtagtgtagcagcccccgcgccgggggctcaggctcaactgagggttttgtcattttcaagtctgaaagtggctgttctcctgcctttgttgtttcttcttttcctggcgtctgggtttttctcccaatggggtgggtggtttgtgtcccgattcactgctagtcccagaaggtgtccagccgagactctttcgggaggaggctcttcgtgctggtactggtgttgtgatcggaacgtgtcgatcccctcttctcatcactgctgctccaactggatttattactccgggaatggtcagagccttggttggagcctaagagaatggaggagggcgtctctctggagccagaaaggtcaagggtcgagccactctccttgcttttctcagctgacgtctccttctctttggaggcgctggccgtttctgaaggtgctgattgtgtgctcgaggagctcccctgggaggacttatttagtgtttctgtgttcacctcagcatccgcttcctgctgaggagcagtagctgactgggtgcaggacttcatgtgctcaggccagtgggcttgctggcaggggtagtcacagtagctggtgttccaacagcagtaaaagatggcctccttcttgcagttggcgcaccactgcttcttcttggtctcatccaccgcctgctgcttctccaactccagctgcttcttcacctcggcgatgagccggtcccgctcctgctccaggctctgccgcatctccgccatggtcagctctaagttgtgtttcatttcggagagctcttgctggtgcagccactggagcttctctatctcgatcctcagcctgcgaatctcagctattgtgcttccagtagtgtttttagaaagatcgttgtatatttctgtcattgttccttttattgcatccatcattttgctagtgtacttggcaatatcagcggcgacatcagctgaggcagtggcgatgggcaggtcagcgttgactgaggacacaagggtgctcatggaccccgagctggtgaccaggggcgatgactgtgtgctggtcaccagggtgatggtggacgtggatgggctctgtgtgatctccttctgctggacagctttcacagcctgtctggtctgatatctcgtcccctgggaagactgaggctgctgctgctggttttgctgctgctgctgctgctgctgacgctgcatcttctgcatgtgccacttttgggaggacgtttgaaacttacttgatgagttccacacgacccgctgcacggccggggcagtctccttcggtaaaagcggcctctgctttttcactgggcttcctgtggcggcgggggccggggccgtgacggtgaccgtggaggacgtgctggtggtggctgtggcgccagccgcggaagtttgggcggaagagcgggtgagcaccggtgtttccgggggagaatggctgcccaccgtcgtggatggtggagttttacctacaacatcctgtttgggagatggttctttgggttccttcttattttttcgaccctcccgcccagaatggtcttctcctaaatctatgacaagttcgctctctgaatcagagtccaggcccaaatggactgttggggaatccgtctcatcttttcccttcagtttatcctttatggggtgaggtgaaggttttgccttttcggaaaagtccttctcaggctcagggctggccttgtccttgactgctccagggtctgccttctcgctggctggtgacgtgcttttcagctcctctttaatctccactgggtttgtaggcttgggcttttttttaacagcagatggctctttgtccatctgacaaccttctttgtcctctgtgtcttctggctcgttcttagacttctgctcatcatcactgatatactcactatcgctactatctgacttctcagaatcctccgaatcgctgtgctctacggccgtatagacatcttccgagatttcatttatgcctaattgtgctttgcaactctctatggtcttgtcaagattcagctggaacctgctacgaatctggcgcttgggagagatgagaggaacaggggtggactgttgctggaccgactcgctcagctccttcaaatccatctcagctttgcttcgatccaggttaagattcaggatgctgccggtggtggaggttttgtccgttttcgtcgtgataggagctgacagttgaggagagaagggctttgggctgccggataaactccctgcttgtcccgtcttggtggaggctggtgaagctgtgctcttatccaggaagtccatggactcctcgctcgcactgaagtggctcgacgtggccttcttctcagcatcctgctccacgtcggagcccgtgtgcacagaagagtttgtgctcatgggggagcgcggcatatccgacaaggaaatccggcggcctgtgcccccactcagcacaggcttgctcatcaggatcttgggggatgccgtcatgtcaaagttgagcttgaccttctcctgcttgtctatcttggcagtgccggcgctggggttggtgggatcgagcagcatttgatactggctgttgggtgtgtagggtgtcctaaatggagagtaattaaaaaccccaaacttcctgcggatgttctccacgtaaacctccatctcttgcatggcactgttgaagatgctcttagtctttttcacagaaaaaggaatttctttagacatgaggtagcaattatttattggaacccaggccctgtcatgttgtccaaagaatcgggcatcgacctgcccgtctttatcccttagagcttttgcaggccagaatggaaaccccttcagtttggcccagaccaaaggatgtggattgctacaaggctcacaaaaccagttatctcgtttttggcaagcagctagataacattctggacatacttcgatttcattcatctcatgttcacagattttgatgactactttcgctatttgcgtcaatttgtgatttcccccattataaatgatgcagttgtgcaaaatccactttgcatcagccaggaaggcttctgtgcagccatacattttctttttcgcattcttttccaatgtacaaaggtccattggatggaagatgtattccgcatagtcagggtgctgttccaatggaacgggcttctggaatgcatctgtccctggctgtttcattttctgaatggcaaacttgagcaggtaggataactgttcaatggtgagcattgtcatggctttactctgggtctcgatgcattctgctactgtaattttctcacattcaggacaaaaccagtccccctctggttccgatgtcagtctcagacacttagcgtgataaacccggggacagagctcacagcaaaggacttggccttcccggtgacaaacccagcagtagaaatcattccgtccatcctgcggtacaacatcaacagggtctgtggtgagtggctgcttcatatagtaaaacggaccatgtcttagttctgactgctccttattgttactgttcagtaagccaggtttctttttctttttaatggggcttgttgatgtgtcctgcggcgagtggccattggaagaatgtggagggctggggaactttcttttctgggctgttctctctgcagagccaggatctttggagcgagtagagatatccatgccctctaccacctcctgttctgtttttatttcctcttcagccaagctccaggatgctttaagccttctgattgttaattctgaggactcagggatggtccgtaattcccaggaatctcatctcctcaacactaaaacaggcagagtcatcggtagctaagctatttatgc

SEQ ID NO: 18770 - RNA, 4503 nt, Homo sapiens
  source 1..4503: mol_type = other RNA
tgagtgtgtgtgtgtgagtgtgtttaaaggaaccacaaagcaaagataaggtttctctttttttcagagttcatgatcctaagactttctgtgttctctcctgtgactgagctgagtggggcttgtttgtttctcttctgtaaacaaggatattgttttttcccttttaggagtagagtcatcatttcaatcacatgaaagaaactagcttctccctgtgtccgtctggtccggagagcttgcgttttaggaacgtggtaacgtagtagctgaaaggagccaacggcttgatgggatagtctgtgccgaaactcccgatcccaacatgctgcgtacagacacacgagcgaaaacggttcgccctcccctgggtatccaaggatgaggacgtgagtatgaaagtggtccccgggcccagtatccattccgtcgtgtgacagacaggctaactgaccatcccttctccaataccaaaacattcttttttgttgttggggttggttgcttttttttttttttttaaatcgtttttctttttctttttttttttttaataagttaaagttaatacaaatataaaaaggggaaagtcctctagattcaatgacatccacaaattgtacattatttacaccaaaagcacagggctcgtgtgggtgaacagtctgcagtcaaagccgatgctgggtgtcctgtagtgtagcagcccccgcgccgggggctcaggctcaactgagggttttgtcattttcaagtctgaaagtggctgttctcctgcctttgttgtttcttcttttcctggcgtctgggtttttctcccaatggggtgggtggtttgtgtcccgattcactgctagtcccagaaggtgtccagccgagactctttcgggaggaggctcttcgtgctggtactggtgttgtgatcggaacgtgtcgatcccctcttctcatcactgctgctccaactggatttattactccgggaatggtcagagccttggttggagcctaagagaatggaggagggcgtctctctggagccagaaaggtcaagggtcgagccactctccttgcttttctcagctgacgtctccttctctttggaggcgctggccgtttctgaaggtgctgattgtgtgctcgaggagctcccctgggaggacttatttagtgtttctgtgttcacctcagcatccgcttcctgctgaggagcagtagctgactgggtgcaggacttcatgtgctcaggccagtgggcttgctggcaggggtagtcacagtagctggtgttccaacagcagtaaaagatggcctccttcttgcagttggcgcaccactgcttcttcttggtctcatccaccgcctgctgcttctccaactccagctgcttcttcacctcggcgatgagccggtcccgctcctgctccaggctctgccgcatctccgccatggtcagctctaagttgtgtttcatttcggagagctcttgctggtgcagccactggagcttctctatctcgatcctcagcctgcgaatctcagctattgtgcttccagtagtgtttttagaaagatcgttgtatatttctgtcattgttccttttattgcatccatcattttgctagtgtacttggcaatatcagcggcgacatcagctgaggcagtggcgatgggcaggtcagcgttgactgaggacacaagggtgctcatggaccccgagctggtgaccaggggcgatgactgtgtgctggtcaccagggtgatggtggacgtggatgggctctgtgtgatctccttctgctggacagctttcacagcctgtctggtctgatatctcgtcccctgggaagactgaggctgctgctgctggttttgctgctgctgctgctgctgctgacgctgcatcttctgcatgtgccacttttgggaggacgtttgaaacttacttgatgagttccacacgacccgctgcacggccggggcagtctccttcggtaaaagcggcctctgctttttcactgggcttcctgtggcggcgggggccggggccgtgacggtgaccgtggaggacgtgctggtggtggctgtggcgccagccgcggaagtttgggcggaagagcgggtgagcaccggtgtttccgggggagaatggctgcccaccgtcgtggatggtggagttttacctacaacatcctgtttgggagatggttctttgggttccttcttattttttcgaccctcccgcccagaatggtcttctcctaaatctatgacaagttcgctctctgaatcagagtccaggcccaaatggactgttggggaatccgtctcatcttttcccttcagtttatcctttatggggtgaggtgaaggttttgccttttcggaaaagtccttctcaggctcagggctggccttgtccttgactgctccagggtctgccttctcgctggctggtgacgtgcttttcagctcctctttaatctccactgggtttgtaggcttgggcttttttttaacagcagatggctctttgtccatctgacaaccttctttgtcctctgtgtcttctggctcgttcttagacttctgctcatcatcactgatatactcactatcgctactatctgacttctcagaatcctccgaatcgctgtgctctacggccgtatagacatcttccgagatttcatttatgcctaattgtgctttgcaactctctatggtcttgtcaagattcagctggaacctgctacgaatctggcgcttgggagagatgagaggaacaggggtggactgttgctggaccgactcgctcagctccttcaaatccatctcagctttgcttcgatccaggttaagattcaggatgctgccggtggtggaggttttgtccgttttcgtcgtgataggagctgacagttgaggagagaagggctttgggctgccggataaactccctgcttgtcccgtcttggtggaggctggtgaagctgtgctcttatccaggaagtccatggactcctcgctcgcactgaagtggctcgacgtggccttcttctcagcatcctgctccacgtcggagcccgtgtgcacagaagagtttgtgctcatgggggagcgcggcatatccgacaaggaaatccggcggcctgtgcccccactcagcacaggcttgctcatcaggatcttgggggatgccgtcatgtcaaagttgagcttgaccttctcctgcttgtctatcttggcagtgccggcgctggggttggtgggatcgagcagcatttgatactggctgttgggtgtgtagggtgtcctaaatggagagtaattaaaaaccccaaacttcctgcggatgttctccacgtaaacctccatctcttgcatggcactgttgaagatgctcttagtctttttcacagaaaaaggaatttctttagacatgaggtagcaattatttattggaacccaggccctgtcatgttgtccaaagaatcgggcatcgacctgcccgtctttatcccttagagcttttgcaggccagaatggaaaccccttcagtttggcccagaccaaaggatgtggattgctacaaggctcacaaaaccagttatctcgtttttggcaagcagctagataacattctggacatacttcgatttcattcatctcatgttcacagattttgatgactactttcgctatttgcgtcaatttgtgatttcccccattataaatgatgcagttgtgcaaaatccactttgcatcagccaggaaggcttctgtgcagccatacattttctttttcgcattcttttccaatgtacaaaggtccattggatggaagatgtattccgcatagtcagggtgctgttccaatggaacgggcttctggaatgcatctgtccctggctgtttcattttctgaatggcaaacttgagcaggtaggataactgttcaatggtgagcattgtcatggctttactctgggtctcgatgcattctgctactgtaattttctcacattcaggacaaaaccagtccccctctggttccgatgtcagtctcagacacttagcgtgataaacccggggacagagctcacagcaaaggacttggccttcccggtgacaaacccagcagtagaaatcattccgtccatcctgcggtacaacatcaacagggtctgtggtgagtggctgcttcatatagtaaaacggaccatgtcttagttctgactgctccttattgttactgttcagtaagccaggtttctttttctttttaatggggcttgttgatgtgtcctgcggcgagtggccattggaagaatgtggagggctggggaactttcttttctgggctgttctctctgcagagccaggatctttggagcgagtagagatatccatgccctctaccacctcctgttctgtttttatttcctcttcagccaagctctgtggatgcattgttaacactgtgtaatgtcaatacttat

SEQ ID NO: 18771 - RNA, 4428 nt, Homo sapiens
  source 1..4428: mol_type = other RNA
tgagtgtgtgtgtgtgagtgtgtttaaaggaaccacaaagcaaagataaggtttctctttttttcagagttcatgatcctaagactttctgtgttctctcctgtgactgagctgagtggggcttgtttgtttctcttctgtaaacaaggatattgttttttcccttttaggagtagagtcatcatttcaatcacatgaaagaaactagcttctccctgtgtccgtctggtccggagagcttgcgttttaggaacgtggtaacgtagtagctgaaaggagccaacggcttgatgggatagtctgtgccgaaactcccgatcccaacatgctgcgtacagacacacgagcgaaaacggttcgccctcccctgggtatccaaggatgaggacgtgagtatgaaagtggtccccgggcccagtatccattccgtcgtgtgacagacaggctaactgaccatcccttctccaataccaaaacattcttttttgttgttggggttggttgcttttttttttttttttaaatcgtttttctttttctttttttttttttaataagttaaagttaatacaaatataaaaaggggaaagtcctctagattcaatgacatccacaaattgtacattatttacaccaaaagcacagggctcgtgtgggtgaacagtctgcagtcaaagccgatgctgggtgtcctgtagtgtagcagcccccgcgccgggggctcaggctcaactgagggttttgtcattttcaagtctgaaagtggctgttctcctgcctttgttgtttcttcttttcctggcgtctgggtttttctcccaatggggtgggtggtttgtgtcccgattcactgctagtcccagaaggtgtccagccgagactctttcgggaggaggctcttcgtgctggtactggtgttgtgatcggaacgtgtcgatcccctcttctcatcactgctgctccaactggatttattactccgggaatggtcagagccttggttggagcctaagagaatggaggagggcgtctctctggagccagaaaggtcaagggtcgagccactctccttgcttttctcagctgacgtctccttctctttggaggcgctggccgtttctgaaggtgctgattgtgtgctcgaggagctcccctgggaggacttatttagtgtttctgtgttcacctcagcatccgcttcctgctgaggagcagtagctgactgggtgcaggacttcatgtgctcaggccagtgggcttgctggcaggggtagtcacagtagctggtgttccaacagcagtaaaagatggcctccttcttgcagttggcgcaccactgcttcttcttggtctcatccaccgcctgctgcttctccaactccagctgcttcttcacctcggcgatgagccggtcccgctcctgctccaggctctgccgcatctccgccatggtcagctctaagttgtgtttcatttcggagagctcttgctggtgcagccactggagcttctctatctcgatcctcagcctgcgaatctcagctattgtgcttccagtagtgtttttagaaagatcgttgtatatttctgtcattgttccttttattgcatccatcattttgctagtgtacttggcaatatcagcggcgacatcagctgaggcagtggcgatgggcaggtcagcgttgactgaggacacaagggtgctcatggaccccgagctggtgaccaggggcgatgactgtgtgctggtcaccagggtgatggtggacgtggatgggctctgtgtgatctccttctgctggacagctttcacagcctgtctggtctgatatctcgtcccctgggaagactgaggctgctgctgctggttttgctgctgctgctgctgctgctgacgctgcatcttctgcatgtgccacttttgggaggacgtttgaaacttacttgatgagttccacacgacccgctgcacggccggggcagtctccttcggtaaaagcggcctctgctttttcactgggcttcctgtggcggcgggggccggggccgtgacggtgaccgtggaggacgtgctggtggtggctgtggcgccagccgcggaagtttgggcggaagagcgggtgagcaccggtgtttccgggggagaatggctgcccaccgtcgtggatggtggagttttacctacaacatcctgtttgggagatggttctttgggttccttcttattttttcgaccctcccgcccagaatggtcttctcctaaatctatgacaagttcgctctctgaatcagagtccaggcccaaatggactgttggggaatccgtctcatcttttcccttcagtttatcctttatggggtgaggtgaaggttttgccttttcggaaaagtccttctcaggctcagggctggccttgtccttgactgctccagggtctgccttctcgctggctggtgacgtgcttttcagctcctctttaatctccactgggtttgtaggcttgggcttttttttaacagcagatggctctttgtccatctgacaaccttctttgtcctctgtgtcttctggctcgttcttagacttctgctcatcatcactgatatactcactatcgctactatctgacttctcagaatcctccgaatcgctgtgctctacggccgtatagacatcttccgagatttcatttatgcctaattgtgctttgcaactctctatggtcttgtcaagattcagctggaacctgctacgaatctggcgcttgggagagatgagaggaacaggggtggactgttgctggaccgactcgctcagctccttcaaatccatctcagctttgcttcgatccaggttaagattcaggatgctgccggtggtggaggttttgtccgttttcgtcgtgataggagctgacagttgaggagagaagggctttgggctgccggataaactccctgcttgtcccgtcttggtggaggctggtgaagctgtgctcttatccaggaagtccatggactcctcgctcgcactgaagtggctcgacgtggccttcttctcagcatcctgctccacgtcggagcccgtgtgcacagaagagtttgtgctcatgggggagcgcggcatatccgacaaggaaatccggcggcctgtgcccccactcagcacaggcttgctcatcaggatcttgggggatgccgtcatgtcaaagttgagcttgaccttctcctgcttgtctatcttggcagtgccggcgctggggttggtgggatcgagcagcatttgatactggctgttgggtgtgtagggtgtcctaaatggagagtaattaaaaaccccaaacttcctgcggatgttctccacgtaaacctccatctcttgcatggcactgttgaagatgctcttagtctttttcacagaaaaaggaatttctttagacatgaggtagcaattatttattggaacccaggccctgtcatgttgtccaaagaatcgggcatcgacctgcccgtctttatcccttagagcttttgcaggccagaatggaaaccccttcagtttggcccagaccaaaggatgtggattgctacaaggctcacaaaaccagttatctcgtttttggcaagcagctagataacattctggacatacttcgatttcattcatctcatgttcacagattttgatgactactttcgctatttgcgtcaatttgtgatttcccccattataaatgatgcagttgtgcaaaatccactttgcatcagccaggaaggcttctgtgcagccatacattttctttttcgcattcttttccaatgtacaaaggtccattggatggaagatgtattccgcatagtcagggtgctgttccaatggaacgggcttctggaatgcatctgtccctggctgtttcattttctgaatggcaaacttgagcaggtaggataactgttcaatggtgagcattgtcatggctttactctgggtctcgatgcattctgctactgtaattttctcacattcaggacaaaaccagtccccctctggttccgatgtcagtctcagacacttagcgtgataaacccggggacagagctcacagcaaaggacttggccttcccggtgacaaacccagcagtagaaatcattccgtccatcctgctccttattgttactgttcagtaagccaggtttctttttctttttaatggggcttgttgatgtgtcctgcggcgagtggccattggaagaatgtggagggctggggaactttcttttctgggctgttctctctgcagagccaggatctttggagcgagtagagatatccatgccctctaccacctcctgttctgtttttatttcctcttcagccaagctctgtggatgcattgttaacactgtgtaatgtcaatacttat

SEQ ID NO: 18772 - RNA, 4627 nt, Homo sapiens
  source 1..4627: mol_type = other RNA
tgagtgtgtgtgtgtgagtgtgtttaaaggaaccacaaagcaaagataaggtttctctttttttcagagttcatgatcctaagactttctgtgttctctcctgtgactgagctgagtggggcttgtttgtttctcttctgtaaacaaggatattgttttttcccttttaggagtagagtcatcatttcaatcacatgaaagaaactagcttctccctgtgtccgtctggtccggagagcttgcgttttaggaacgtggtaacgtagtagctgaaaggagccaacggcttgatgggatagtctgtgccgaaactcccgatcccaacatgctgcgtacagacacacgagcgaaaacggttcgccctcccctgggtatccaaggatgaggacgtgagtatgaaagtggtccccgggcccagtatccattccgtcgtgtgacagacaggctaactgaccatcccttctccaataccaaaacattcttttttgttgttggggttggttgcttttttttttttttttaaatcgtttttctttttctttttttttttttaataagttaaagttaatacaaatataaaaaggggaaagtcctctagattcaatgacatccacaaattgtacattatttacaccaaaagcacagggctcgtgtgggtgaacagtctgcagtcaaagccgatgctgggtgtcctgtagtgtagcagcccccgcgccgggggctcaggctcaactgagggttttgtcattttcaagtctgaaagtggctgttctcctgcctttgttgtttcttcttttcctggcgtctgggtttttctcccaatggggtgggtggtttgtgtcccgattcactgctagtcccagaaggtgtccagccgagactctttcgggaggaggctcttcgtgctggtactggtgttgtgatcggaacgtgtcgatcccctcttctcatcactgctgctccaactggatttattactccgggaatggtcagagccttggttggagcctaagagaatggaggagggcgtctctctggagccagaaaggtcaagggtcgagccactctccttgcttttctcagctgacgtctccttctctttggaggcgctggccgtttctgaaggtgctgattgtgtgctcgaggagctcccctgggaggacttatttagtgtttctgtgttcacctcagcatccgcttcctgctgaggagcagtagctgactgggtgcaggacttcatgtgctcaggccagtgggcttgctggcaggggtagtcacagtagctggtgttccaacagcagtaaaagatggcctccttcttgcagttggcgcaccactgcttcttcttggtctcatccaccgcctgctgcttctccaactccagctgcttcttcacctcggcgatgagccggtcccgctcctgctccaggctctgccgcatctccgccatggtcagctctaagttgtgtttcatttcggagagctcttgctggtgcagccactggagcttctctatctcgatcctcagcctgcgaatctcagctattgtgcttccagtagtgtttttagaaagatcgttgtatatttctgtcattgttccttttattgcatccatcattttgctagtgtacttggcaatatcagcggcgacatcagctgaggcagtggcgatgggcaggtcagcgttgactgaggacacaagggtgctcatggaccccgagctggtgaccaggggcgatgactgtgtgctggtcaccagggtgatggtggacgtggatgggctctgtgtgatctccttctgctggacagctttcacagcctgtctggtctgatatctcgtcccctgggaagactgaggctgctgctgctggttttgctgctgctgctgctgctgctgacgctgcatcttctgcatgtgccacttttgggaggacgtttgaaacttacttgatgagttccacacgacccgctgcacggccggggcagtctccttcggtaaaagcggcctctgctttttcactgggcttcctgtggcggcgggggccggggccgtgacggtgaccgtggaggacgtgctggtggtggctgtggcgccagccgcggaagtttgggcggaagagcgggtgagcaccggtgtttccgggggagaatggctgcccaccgtcgtggatggtggagttttacctacaacatcctgtttgggagatggttctttgggttccttcttattttttcgaccctcccgcccagaatggtcttctcctaaatctatgacaagttcgctctctgaatcagagtccaggcccaaatggactgttggggaatccgtctcatcttttcccttcagtttatcctttatggggtgaggtgaaggttttgccttttcggaaaagtccttctcaggctcagggctggccttgtccttgactgctccagggtctgccttctcgctggctggtgacgtgcttttcagctcctctttaatctccactgggtttgtaggcttgggcttttttttaacagcagatggctctttgtccatctgacaaccttctttgtcctctgtgtcttctggctcgttcttagacttctgctcatcatcactgatatactcactatcgctactatctgacttctcagaatcctccgaatcgctgtgctctacggccgtatagacatcttccgagatttcatttatgcctaattgtgctttgcaactctctatggtcttgtcaagattcagctggaacctgctacgaatctggcgcttgggagagatgagaggaacaggggtggactgttgctggaccgactcgctcagctccttcaaatccatctcagctttgcttcgatccaggttaagattcaggatgctgccggtggtggaggttttgtccgttttcgtcgtgataggagctgacagttgaggagagaagggctttgggctgccggataaactccctgcttgtcccgtcttggtggaggctggtgaagctgtgctcttatccaggaagtccatggactcctcgctcgcactgaagtggctcgacgtggccttcttctcagcatcctgctccacgtcggagcccgtgtgcacagaagagtttgtgctcatgggggagcgcggcatatccgacaaggaaatccggcggcctgtgcccccactcagcacaggcttgctcatcaggatcttgggggatgccgtcatgtcaaagttgagcttgaccttctcctgcttgtctatcttggcagtgccggcgctggggttggtgggatcgagcagcatttgatactggctgttgggtgtgtagggtgtcctaaatggagagtaattaaaaaccccaaacttcctgcggatgttctccacgtaaacctccatctcttgcatggcactgttgaagatgctcttagtctttttcacagaaaaaggaatttctttagacatgaggtagcaattatttattggaacccaggccctgtcatgttgtccaaagaatcgggcatcgacctgcccgtctttatcccttagagcttttgcaggccagaatggaaaccccttcagtttggcccagaccaaaggatgtggattgctacaaggctcacaaaaccagttatctcgtttttggcaagcagctagataacattctggacatacttcgatttcattcatctcatgttcacagattttgatgactactttcgctatttgcgtcaatttgtgatttcccccattataaatgatgcagttgtgcaaaatccactttgcatcagccaggaaggcttctgtgcagccatacattttctttttcgcattcttttccaatgtacaaaggtccattggatggaagatgtattccgcatagtcagggtgctgttccaatggaacgggcttctggaatgcatctgtccctggctgtttcattttctgaatggcaaacttgagcaggtaggataactgttcaatggtgagcattgtcatggctttactctgggtctcgatgcattctgctactgtaattttctcacattcaggacaaaaccagtccccctctggttccgatgtcagtctcagacacttagcgtgataaacccggggacagagctcacagcaaaggacttggccttcccggtgacaaacccagcagtagaaatcattccgtccatcctgctccttattgttactgttcagtaagccaggtttctttttctttttaatggggcttgttgatgtgtcctgcggcgagtggccattggaagaatgtggagggctggggaactttcttttctgggctgttctctctgcagagccaggatctttggagcgagtagagatatccatgccctctaccacctcctgttctgtttttatttcctcttcagccaagttgaaggatttctgcagcgatgaaaacattcaaaggtgtattgatcatggaggaaggctgcattcaagggaaccattatttggcttgtaacagcctagaggagctgaatacttcaggcaggaatgctgccaacaaatgttcaagcaaccgtctcatttttccacagttaggaagagagaacaggctggcagatttgggactctgtggatgcattgttaacactgtgtaatgtcaatacttat

SEQ ID NO: 18773 - RNA, 4287 nt, Homo sapiens
  source 1..4287: mol_type = other RNA
tgagtgtgtgtgtgtgagtgtgtttaaaggaaccacaaagcaaagataaggtttctctttttttcagagttcatgatcctaagactttctgtgttctctcctgtgactgagctgagtggggcttgtttgtttctcttctgtaaacaaggatattgttttttcccttttaggagtagagtcatcatttcaatcacatgaaagaaactagcttctccctgtgtccgtctggtccggagagcttgcgttttaggaacgtggtaacgtagtagctgaaaggagccaacggcttgatgggatagtctgtgccgaaactcccgatcccaacatgctgcgtacagacacacgagcgaaaacggttcgccctcccctgggtatccaaggatgaggacgtgagtatgaaagtggtccccgggcccagtatccattccgtcgtgtgacagacaggctaactgaccatcccttctccaataccaaaacattcttttttgttgttggggttggttgcttttttttttttttttaaatcgtttttctttttctttttttttttttaataagttaaagttaatacaaatataaaaaggggaaagtcctctagattcaatgacatccacaaattgtacattatttacaccaaaagcacagggctcgtgtgggtgaacagtctgcagtcaaagccgatgctgggtgtcctgtagtgtagcagcccccgcgccgggggctcaggctcaactgagggttttgtcattttcaagtctgaaagtggctgttctcctgcctttgttgtttcttcttttcctggcgtctgggtttttctcccaatggggtgggtggtttgtgtcccgattcactgctagtcccagaaggtgtccagccgagactctttcgggaggaggctcttcgtgctggtactggtgttgtgatcggaacgtgtcgatcccctcttctcatcactgctgctccaactggatttattactccgggaatggtcagagccttggttggagcctaagagaatggaggagggcgtctctctggagccagaaaggtcaagggtcgagccactctccttgcttttctcagctgacgtctccttctctttggaggcgctggccgtttctgaaggtgctgattgtgtgctcgaggagctcccctgggaggacttatttagtgtttctgtgttcacctcagcatccgcttcctgctgaggagcagtagctgactgggtgcaggacttcatgtgctcaggccagtgggcttgctggcaggggtagtcacagtagctggtgttccaacagcagtaaaagatggcctccttcttgcagttggcgcaccactgcttcttcttggtctcatccaccgcctgctgcttctccaactccagctgcttcttcacctcggcgatgagccggtcccgctcctgctccaggctctgccgcatctccgccatggtcagctctaagttgtgtttcatttcggagagctcttgctggtgcagccactggagcttctctatctcgatcctcagcctgcgaatctcagctattgtgcttccagtagtgtttttagaaagatcgttgtatatttctgtcattgttccttttattgcatccatcattttgctagtgtacttggcaatatcagcggcgacatcagctgaggcagtggcgatgggcaggtcagcgttgactgaggacacaagggtgctcatggaccccgagctggtgaccaggggcgatgactgtgtgctggtcaccagggtgatggtggacgtggatgggctctgtgtgatctccttctgctggacagctttcacagcctgtctggtctgatatctcgtcccctgggaagactgaggctgctgctgctggttttgctgctgctgctgctgctgctgacgctgcatcttctgcatgtgccacttttgggaggacgtttgaaacttacttgatgagttccacacgacccgctgcacggccggggcagtctccttcggtaaaagcggcctctgctttttcactgggcttcctgtggcggcgggggccggggccgtgacggtgaccgtggaggacgtgctggtggtggctgtggcgccagccgcggaagtttgggcggaagagcgggtgagcaccggtgtttccgggggagaatggctgcccaccgtcgtggatggtggagttttacctacaacatcctgtttgggagatggttctttgggttccttcttattttttcgaccctcccgcccagaatggtcttctcctaaatctatgacaagttcgctctctgaatcagagtccaggcccaaatggactgttggggaatccgtctcatcttttcccttcagtttatcctttatggggtgaggtgaaggttttgccttttcggaaaagtccttctcaggctcagggctggccttgtccttgactgctccagggtctgccttctcgctggctggtgacgtgcttttcagctcctctttaatctccactgggtttgtaggcttgggcttttttttaacagcagatggctctttgtccatctgacaaccttctttgtcctctgtgtcttctggctcgttcttagacttctgctcatcatcactgatatactcactatcgctactatctgacttctcagaatcctccgaatcgctgtgctctacggccgtatagacatcttccgagatttcatttatgcctaattgtgctttgcaactctctatggtcttgtcaagattcagctggaacctgctacgaatctggcgcttgggagagatgagaggaacaggggtggactgttgctggaccgactcgctcagctccttcaaatccatctcagctttgcttcgatctgtgctcttatccaggaagtccatggactcctcgctcgcactgaagtggctcgacgtggccttcttctcagcatcctgctccacgtcggagcccgtgtgcacagaagagtttgtgctcatgggggagcgcggcatatccgacaaggaaatccggcggcctgtgcccccactcagcacaggcttgctcatcaggatcttgggggatgccgtcatgtcaaagttgagcttgaccttctcctgcttgtctatcttggcagtgccggcgctggggttggtgggatcgagcagcatttgatactggctgttgggtgtgtagggtgtcctaaatggagagtaattaaaaaccccaaacttcctgcggatgttctccacgtaaacctccatctcttgcatggcactgttgaagatgctcttagtctttttcacagaaaaaggaatttctttagacatgaggtagcaattatttattggaacccaggccctgtcatgttgtccaaagaatcgggcatcgacctgcccgtctttatcccttagagcttttgcaggccagaatggaaaccccttcagtttggcccagaccaaaggatgtggattgctacaaggctcacaaaaccagttatctcgtttttggcaagcagctagataacattctggacatacttcgatttcattcatctcatgttcacagattttgatgactactttcgctatttgcgtcaatttgtgatttcccccattataaatgatgcagttgtgcaaaatccactttgcatcagccaggaaggcttctgtgcagccatacattttctttttcgcattcttttccaatgtacaaaggtccattggatggaagatgtattccgcatagtcagggtgctgttccaatggaacgggcttctggaatgcatctgtccctggctgtttcattttctgaatggcaaacttgagcaggtaggataactgttcaatggtgagcattgtcatggctttactctgggtctcgatgcattctgctactgtaattttctcacattcaggacaaaaccagtccccctctggttccgatgtcagtctcagacacttagcgtgataaacccggggacagagctcacagcaaaggacttggccttcccggtgacaaacccagcagtagaaatcattccgtccatcctgctccttattgttactgttcagtaagccaggtttctttttctttttaatggggcttgttgatgtgtcctgcggcgagtggccattggaagaatgtggagggctggggaactttcttttctgggctgttctctctgcagagccaggatctttggagcgagtagagatatccatgccctctaccacctcctgttctgtttttatttcctcttcagccaagctctgtggatgcattgttaacactgtgtaatgtcaatacttat

SEQ ID NO: 18774 - RNA, 4365 nt, Homo sapiens
  source 1..4365: mol_type = other RNA
tgagtgtgtgtgtgtgagtgtgtttaaaggaaccacaaagcaaagataaggtttctctttttttcagagttcatgatcctaagactttctgtgttctctcctgtgactgagctgagtggggcttgtttgtttctcttctgtaaacaaggatattgttttttcccttttaggagtagagtcatcatttcaatcacatgaaagaaactagcttctccctgtgtccgtctggtccggagagcttgcgttttaggaacgtggtaacgtagtagctgaaaggagccaacggcttgatgggatagtctgtgccgaaactcccgatcccaacatgctgcgtacagacacacgagcgaaaacggttcgccctcccctgggtatccaaggatgaggacgtgagtatgaaagtggtccccgggcccagtatccattccgtcgtgtgacagacaggctaactgaccatcccttctccaataccaaaacattcttttttgttgttggggttggttgcttttttttttttttttaaatcgtttttctttttctttttttttttttaataagttaaagttaatacaaatataaaaaggggaaagtcctctagattcaatgacatccacaaattgtacattatttacaccaaaagcacagggctcgtgtgggtgaacagtctgcagtcaaagccgatgctgggtgtcctgtagtgtagcagcccccgcgccgggggctcaggctcaactgagggttttgtcattttcaagtctgaaagtggctgttctcctgcctttgttgtttcttcttttcctggcgtctgggtttttctcccaatggggtgggtggtttgtgtcccgattcactgctagtcccagaaggtgtccagccgagactctttcgggaggaggctcttcgtgctggtactggtgttgtgatcggaacgtgtcgatcccctcttctcatcactgctgctccaactggatttattactccgggaatggtcagagccttggttggagcctaagagaatggaggagggcgtctctctggagccagaaaggtcaagggtcgagccactctccttgcttttctcagctgacgtctccttctctttggaggcgctggccgtttctgaaggtgctgattgtgtgctcgaggagctcccctgggaggacttatttagtgtttctgtgttcacctcagcatccgcttcctgctgaggagcagtagctgactgggtgcaggacttcatgtgctcaggccagtgggcttgctggcaggggtagtcacagtagctggtgttccaacagcagtaaaagatggcctccttcttgcagttggcgcaccactgcttcttcttggtctcatccaccgcctgctgcttctccaactccagctgcttcttcacctcggcgatgagccggtcccgctcctgctccaggctctgccgcatctccgccatggtcagctctaagttgtgtttcatttcggagagctcttgctggtgcagccactggagcttctctatctcgatcctcagcctgcgaatctcagctattgtgcttccagtagtgtttttagaaagatcgttgtatatttctgtcattgttccttttattgcatccatcattttgctagtgtacttggcaatatcagcggcgacatcagctgaggcagtggcgatgggcaggtcagcgttgactgaggacacaagggtgctcatggaccccgagctggtgaccaggggcgatgactgtgtgctggtcaccagggtgatggtggacgtggatgggctctgtgtgatctccttctgctggacagttgatgagttccacacgacccgctgcacggccggggcagtctccttcggtaaaagcggcctctgctttttcactgggcttcctgtggcggcgggggccggggccgtgacggtgaccgtggaggacgtgctggtggtggctgtggcgccagccgcggaagtttgggcggaagagcgggtgagcaccggtgtttccgggggagaatggctgcccaccgtcgtggatggtggagttttacctacaacatcctgtttgggagatggttctttgggttccttcttattttttcgaccctcccgcccagaatggtcttctcctaaatctatgacaagttcgctctctgaatcagagtccaggcccaaatggactgttggggaatccgtctcatcttttcccttcagtttatcctttatggggtgaggtgaaggttttgccttttcggaaaagtccttctcaggctcagggctggccttgtccttgactgctccagggtctgccttctcgctggctggtgacgtgcttttcagctcctctttaatctccactgggtttgtaggcttgggcttttttttaacagcagatggctctttgtccatctgacaaccttctttgtcctctgtgtcttctggctcgttcttagacttctgctcatcatcactgatatactcactatcgctactatctgacttctcagaatcctccgaatcgctgtgctctacggccgtatagacatcttccgagatttcatttatgcctaattgtgctttgcaactctctatggtcttgtcaagattcagctggaacctgctacgaatctggcgcttgggagagatgagaggaacaggggtggactgttgctggaccgactcgctcagctccttcaaatccatctcagctttgcttcgatccaggttaagattcaggatgctgccggtggtggaggttttgtccgttttcgtcgtgataggagctgacagttgaggagagaagggctttgggctgccggataaactccctgcttgtcccgtcttggtggaggctggtgaagctgtgctcttatccaggaagtccatggactcctcgctcgcactgaagtggctcgacgtggccttcttctcagcatcctgctccacgtcggagcccgtgtgcacagaagagtttgtgctcatgggggagcgcggcatatccgacaaggaaatccggcggcctgtgcccccactcagcacaggcttgctcatcaggatcttgggggatgccgtcatgtcaaagttgagcttgaccttctcctgcttgtctatcttggcagtgccggcgctggggttggtgggatcgagcagcatttgatactggctgttgggtgtgtagggtgtcctaaatggagagtaattaaaaaccccaaacttcctgcggatgttctccacgtaaacctccatctcttgcatggcactgttgaagatgctcttagtctttttcacagaaaaaggaatttctttagacatgaggtagcaattatttattggaacccaggccctgtcatgttgtccaaagaatcgggcatcgacctgcccgtctttatcccttagagcttttgcaggccagaatggaaaccccttcagtttggcccagaccaaaggatgtggattgctacaaggctcacaaaaccagttatctcgtttttggcaagcagctagataacattctggacatacttcgatttcattcatctcatgttcacagattttgatgactactttcgctatttgcgtcaatttgtgatttcccccattataaatgatgcagttgtgcaaaatccactttgcatcagccaggaaggcttctgtgcagccatacattttctttttcgcattcttttccaatgtacaaaggtccattggatggaagatgtattccgcatagtcagggtgctgttccaatggaacgggcttctggaatgcatctgtccctggctgtttcattttctgaatggcaaacttgagcaggtaggataactgttcaatggtgagcattgtcatggctttactctgggtctcgatgcattctgctactgtaattttctcacattcaggacaaaaccagtccccctctggttccgatgtcagtctcagacacttagcgtgataaacccggggacagagctcacagcaaaggacttggccttcccggtgacaaacccagcagtagaaatcattccgtccatcctgcggtacaacatcaacagggtctgtggtgagtggctgcttcatatagtaaaacggaccatgtcttagttctgactgctccttattgttactgttcagtaagccaggtttctttttctttttaatggggcttgttgatgtgtcctgcggcgagtggccattggaagaatgtggagggctggggaactttcttttctgggctgttctctctgcagagccaggatctttggagcgagtagagatatccatgccctctaccacctcctgttctgtttttatttcctcttcagccaagctctgtggatgcattgttaacactgtgtaatgtcaatacttat

SEQ ID NO: 18775 - RNA, 4290 nt, Homo sapiens
  source 1..4290: mol_type = other RNA
tgagtgtgtgtgtgtgagtgtgtttaaaggaaccacaaagcaaagataaggtttctctttttttcagagttcatgatcctaagactttctgtgttctctcctgtgactgagctgagtggggcttgtttgtttctcttctgtaaacaaggatattgttttttcccttttaggagtagagtcatcatttcaatcacatgaaagaaactagcttctccctgtgtccgtctggtccggagagcttgcgttttaggaacgtggtaacgtagtagctgaaaggagccaacggcttgatgggatagtctgtgccgaaactcccgatcccaacatgctgcgtacagacacacgagcgaaaacggttcgccctcccctgggtatccaaggatgaggacgtgagtatgaaagtggtccccgggcccagtatccattccgtcgtgtgacagacaggctaactgaccatcccttctccaataccaaaacattcttttttgttgttggggttggttgcttttttttttttttttaaatcgtttttctttttctttttttttttttaataagttaaagttaatacaaatataaaaaggggaaagtcctctagattcaatgacatccacaaattgtacattatttacaccaaaagcacagggctcgtgtgggtgaacagtctgcagtcaaagccgatgctgggtgtcctgtagtgtagcagcccccgcgccgggggctcaggctcaactgagggttttgtcattttcaagtctgaaagtggctgttctcctgcctttgttgtttcttcttttcctggcgtctgggtttttctcccaatggggtgggtggtttgtgtcccgattcactgctagtcccagaaggtgtccagccgagactctttcgggaggaggctcttcgtgctggtactggtgttgtgatcggaacgtgtcgatcccctcttctcatcactgctgctccaactggatttattactccgggaatggtcagagccttggttggagcctaagagaatggaggagggcgtctctctggagccagaaaggtcaagggtcgagccactctccttgcttttctcagctgacgtctccttctctttggaggcgctggccgtttctgaaggtgctgattgtgtgctcgaggagctcccctgggaggacttatttagtgtttctgtgttcacctcagcatccgcttcctgctgaggagcagtagctgactgggtgcaggacttcatgtgctcaggccagtgggcttgctggcaggggtagtcacagtagctggtgttccaacagcagtaaaagatggcctccttcttgcagttggcgcaccactgcttcttcttggtctcatccaccgcctgctgcttctccaactccagctgcttcttcacctcggcgatgagccggtcccgctcctgctccaggctctgccgcatctccgccatggtcagctctaagttgtgtttcatttcggagagctcttgctggtgcagccactggagcttctctatctcgatcctcagcctgcgaatctcagctattgtgcttccagtagtgtttttagaaagatcgttgtatatttctgtcattgttccttttattgcatccatcattttgctagtgtacttggcaatatcagcggcgacatcagctgaggcagtggcgatgggcaggtcagcgttgactgaggacacaagggtgctcatggaccccgagctggtgaccaggggcgatgactgtgtgctggtcaccagggtgatggtggacgtggatgggctctgtgtgatctccttctgctggacagttgatgagttccacacgacccgctgcacggccggggcagtctccttcggtaaaagcggcctctgctttttcactgggcttcctgtggcggcgggggccggggccgtgacggtgaccgtggaggacgtgctggtggtggctgtggcgccagccgcggaagtttgggcggaagagcgggtgagcaccggtgtttccgggggagaatggctgcccaccgtcgtggatggtggagttttacctacaacatcctgtttgggagatggttctttgggttccttcttattttttcgaccctcccgcccagaatggtcttctcctaaatctatgacaagttcgctctctgaatcagagtccaggcccaaatggactgttggggaatccgtctcatcttttcccttcagtttatcctttatggggtgaggtgaaggttttgccttttcggaaaagtccttctcaggctcagggctggccttgtccttgactgctccagggtctgccttctcgctggctggtgacgtgcttttcagctcctctttaatctccactgggtttgtaggcttgggcttttttttaacagcagatggctctttgtccatctgacaaccttctttgtcctctgtgtcttctggctcgttcttagacttctgctcatcatcactgatatactcactatcgctactatctgacttctcagaatcctccgaatcgctgtgctctacggccgtatagacatcttccgagatttcatttatgcctaattgtgctttgcaactctctatggtcttgtcaagattcagctggaacctgctacgaatctggcgcttgggagagatgagaggaacaggggtggactgttgctggaccgactcgctcagctccttcaaatccatctcagctttgcttcgatccaggttaagattcaggatgctgccggtggtggaggttttgtccgttttcgtcgtgataggagctgacagttgaggagagaagggctttgggctgccggataaactccctgcttgtcccgtcttggtggaggctggtgaagctgtgctcttatccaggaagtccatggactcctcgctcgcactgaagtggctcgacgtggccttcttctcagcatcctgctccacgtcggagcccgtgtgcacagaagagtttgtgctcatgggggagcgcggcatatccgacaaggaaatccggcggcctgtgcccccactcagcacaggcttgctcatcaggatcttgggggatgccgtcatgtcaaagttgagcttgaccttctcctgcttgtctatcttggcagtgccggcgctggggttggtgggatcgagcagcatttgatactggctgttgggtgtgtagggtgtcctaaatggagagtaattaaaaaccccaaacttcctgcggatgttctccacgtaaacctccatctcttgcatggcactgttgaagatgctcttagtctttttcacagaaaaaggaatttctttagacatgaggtagcaattatttattggaacccaggccctgtcatgttgtccaaagaatcgggcatcgacctgcccgtctttatcccttagagcttttgcaggccagaatggaaaccccttcagtttggcccagaccaaaggatgtggattgctacaaggctcacaaaaccagttatctcgtttttggcaagcagctagataacattctggacatacttcgatttcattcatctcatgttcacagattttgatgactactttcgctatttgcgtcaatttgtgatttcccccattataaatgatgcagttgtgcaaaatccactttgcatcagccaggaaggcttctgtgcagccatacattttctttttcgcattcttttccaatgtacaaaggtccattggatggaagatgtattccgcatagtcagggtgctgttccaatggaacgggcttctggaatgcatctgtccctggctgtttcattttctgaatggcaaacttgagcaggtaggataactgttcaatggtgagcattgtcatggctttactctgggtctcgatgcattctgctactgtaattttctcacattcaggacaaaaccagtccccctctggttccgatgtcagtctcagacacttagcgtgataaacccggggacagagctcacagcaaaggacttggccttcccggtgacaaacccagcagtagaaatcattccgtccatcctgctccttattgttactgttcagtaagccaggtttctttttctttttaatggggcttgttgatgtgtcctgcggcgagtggccattggaagaatgtggagggctggggaactttcttttctgggctgttctctctgcagagccaggatctttggagcgagtagagatatccatgccctctaccacctcctgttctgtttttatttcctcttcagccaagctctgtggatgcattgttaacactgtgtaatgtcaatacttat

SEQ ID NO: 18776 - RNA, 4496 nt, Homo sapiens
  source 1..4496: mol_type = other RNA
tgagtgtgtgtgtgtgagtgtgtttaaaggaaccacaaagcaaagataaggtttctctttttttcagagttcatgatcctaagactttctgtgttctctcctgtgactgagctgagtggggcttgtttgtttctcttctgtaaacaaggatattgttttttcccttttaggagtagagtcatcatttcaatcacatgaaagaaactagcttctccctgtgtccgtctggtccggagagcttgcgttttaggaacgtggtaacgtagtagctgaaaggagccaacggcttgatgggatagtctgtgccgaaactcccgatcccaacatgctgcgtacagacacacgagcgaaaacggttcgccctcccctgggtatccaaggatgaggacgtgagtatgaaagtggtccccgggcccagtatccattccgtcgtgtgacagacaggctaactgaccatcccttctccaataccaaaacattcttttttgttgttggggttggttgcttttttttttttttttaaatcgtttttctttttctttttttttttttaataagttaaagttaatacaaatataaaaaggggaaagtcctctagattcaatgacatccacaaattgtacattatttacaccaaaagcacagggctcgtgtgggtgaacagtctgcagtcaaagccgatgctgggtgtcctgtagtgtagcagcccccgcgccgggggctcaggctcaactgagggttttgtcattttcaagtctgaaagtggctgttctcctgcctttgttgtttcttcttttcctggcgtctgggtttttctcccaatggggtgggtggtttgtgtcccgattcactgctagtcccagaaggtgtccagccgagactctttcgggaggaggctcttcgtgctggtactggtgttgtgatcggaacgtgtcgatcccctcttctcatcactgctgctccaactggatttattactccgggaatggtcagagccttggttggagcctaagagaatggaggagggcgtctctctggagccagaaaggtcaagggtcgagccactctccttgcttttctcagctgacgtctccttctctttggaggcgctggccgtttctgaaggtgctgattgtgtgctcgaggagctcccctgggaggacttatttagtgtttctgtgttcacctcagcatccgcttcctgctgaggagcagtagctgactgggtgcaggacttcatgtgctcaggccagtgggcttgctggcaggggtagtcacagtagctggtgttccaacagcagtaaaagatggcctccttcttgcagttggcgcaccactgcttcttcttggtctcatccaccgcctgctgcttctccaactccagctgcttcttcacctcggcgatgagccggtcccgctcctgctccaggctctgccgcatctccgccatggtcagctctaagttgtgtttcatttcggagagctcttgctggtgcagccactggagcttctctatctcgatcctcagcctgcgaatctcagctattgtgcttccagtagtgtttttagaaagatcgttgtatatttctgtcattgttccttttattgcatccatcattttgctagtgtacttggcaatatcagcggcgacatcagctgaggcagtggcgatgggcaggtcagcgttgactgaggacacaagggtgctcatggaccccgagctggtgaccaggggcgatgactgtgtgctggtcaccagggtgatggtggacgtggatgggctctgtgtgatctccttctgctggacagttgatgagttccacacgacccgctgcacggccggggcagtctccttcggtaaaagcggcctctgctttttcactgggcttcctgtggcggcgggggccggggccgtgacggtgaccgtggaggacgtgctggtggtggctgtggcgccagccgcggaagtttgggcggaagagcgggtgagcaccggtgtttccgggggagaatggctgcccaccgtcgtggatggtggagttttacctacaacatcctgtttgggagatggttctttgggttccttcttattttttcgaccctcccgcccagaatggtcttctcctaaatctatgacaagttcgctctctgaatcagagtccaggcccaaatggactgttggggaatccgtctcatcttttcccttcagtttatcctttatggggtgaggtgaaggttttgccttttcggaaaagtccttctcaggctcagggctggccttgtccttgactgctccagggtctgccttctcgctggctggtgacgtgcttttcagctcctctttaatctccactgggtttgtaggcttgggcttttttttaacagcagatggctctttgtccatctgacaaccttctttgtcctctgtgtcttctggctcgttcttagacttctgctcatcatcactgatatactcactatcgctactatctgacttctcagaatcctccgaatcgctgtgctctacggccgtatagacatcttccgagatttcatttatgcctaattgtgctttgcaactctctatggtcttgtcaagattcagctggaacctgctacgaatctggcgcttgggagagatgagaggaacaggggtggactgttgctggaccgactcgctcagctccttcaaatccatctcagctttgcttcgatccaggttaagattcaggatgctgccggtggtggaggttttgtccgttttcgtcgtgataggagctgacagttgaggagagaagggctttgggctgccggataaactccctgcttgtcccgtcttggtggaggctggtgaagctgtgctcttatccaggaagtccatggactcctcgctcgcactgaagtggctcgacgtggccttcttctcagcatcctgctccacgtcggagcccgtgtgcacagaagagtttgtgctcatgggggagcgcggcatatccgacaaggaaatccggcggcctgtgcccccactcagcacaggcttgctcatcaggatcttgggggatgccgtcatgtcaaagttgagcttgaccttctcctgcttgtctatcttggcagtgccggcgctggggttggtgggatcgagcagcatttgatactggctgttgggtgtgtagggtgtcctaaatggagagtaattaaaaaccccaaacttcctgcggatgttctccacgtaaacctccatctcttgcatggcactgttgaagatgctcttagtctttttcacagaaaaaggaatttctttagacatgaggtagcaattatttattggaacccaggccctgtcatgttgtccaaagaatcgggcatcgacctgcccgtctttatcccttagagcttttgcaggccagaatggaaaccccttcagtttggcccagaccaaaggatgtggattgctacaaggctcacaaaaccagttatctcgtttttggcaagcagctagataacattctggacatacttcgatttcattcatcttgttacttaagatgctgataaaactgggtactatttaatgacaagaggagtaattaaatgaatgtccatgtgttgtatgtaatactatacagccatgaaaaattctgttcttcctacgagtttaattacctcatgttcacagattttgatgactactttcgctatttgcgtcaatttgtgatttcccccattataaatgatgcagttgtgcaaaatccactttgcatcagccaggaaggcttctgtgcagccatacattttctttttcgcattcttttccaatgtacaaaggtccattggatggaagatgtattccgcatagtcagggtgctgttccaatggaacgggcttctggaatgcatctgtccctggctgtttcattttctgaatggcaaacttgagcaggtaggataactgttcaatggtgagcattgtcatggctttactctgggtctcgatgcattctgctactgtaattttctcacattcaggacaaaaccagtccccctctggttccgatgtcagtctcagacacttagcgtgataaacccggggacagagctcacagcaaaggacttggccttcccggtgacaaacccagcagtagaaatcattccgtccatcctgcggtacaacatcaacagggtctgtggtgagtggctgcttcatatagtaaaacggaccatgtcttagttctgactgctccttattgttactgttcagtaagccaggtttctttttctttttaatggggcttgttgatgtgtcctgcggcgagtggccattggaagaatgtggagggctggggaactttcttttctgggctgttctctctgcagagccaggatctttggagcgagtagagatatccatgccctctaccacctcctgttctgtttttatttcctcttcagccaagctctgtggatgcattgttaacactgtgtaatgtcaatacttat

SEQ ID NO: 18777 - RNA, 4149 nt, Homo sapiens
  source 1..4149: mol_type = other RNA
tgagtgtgtgtgtgtgagtgtgtttaaaggaaccacaaagcaaagataaggtttctctttttttcagagttcatgatcctaagactttctgtgttctctcctgtgactgagctgagtggggcttgtttgtttctcttctgtaaacaaggatattgttttttcccttttaggagtagagtcatcatttcaatcacatgaaagaaactagcttctccctgtgtccgtctggtccggagagcttgcgttttaggaacgtggtaacgtagtagctgaaaggagccaacggcttgatgggatagtctgtgccgaaactcccgatcccaacatgctgcgtacagacacacgagcgaaaacggttcgccctcccctgggtatccaaggatgaggacgtgagtatgaaagtggtccccgggcccagtatccattccgtcgtgtgacagacaggctaactgaccatcccttctccaataccaaaacattcttttttgttgttggggttggttgcttttttttttttttttaaatcgtttttctttttctttttttttttttaataagttaaagttaatacaaatataaaaaggggaaagtcctctagattcaatgacatccacaaattgtacattatttacaccaaaagcacagggctcgtgtgggtgaacagtctgcagtcaaagccgatgctgggtgtcctgtagtgtagcagcccccgcgccgggggctcaggctcaactgagggttttgtcattttcaagtctgaaagtggctgttctcctgcctttgttgtttcttcttttcctggcgtctgggtttttctcccaatggggtgggtggtttgtgtcccgattcactgctagtcccagaaggtgtccagccgagactctttcgggaggaggctcttcgtgctggtactggtgttgtgatcggaacgtgtcgatcccctcttctcatcactgctgctccaactggatttattactccgggaatggtcagagccttggttggagcctaagagaatggaggagggcgtctctctggagccagaaaggtcaagggtcgagccactctccttgcttttctcagctgacgtctccttctctttggaggcgctggccgtttctgaaggtgctgattgtgtgctcgaggagctcccctgggaggacttatttagtgtttctgtgttcacctcagcatccgcttcctgctgaggagcagtagctgactgggtgcaggacttcatgtgctcaggccagtgggcttgctggcaggggtagtcacagtagctggtgttccaacagcagtaaaagatggcctccttcttgcagttggcgcaccactgcttcttcttggtctcatccaccgcctgctgcttctccaactccagctgcttcttcacctcggcgatgagccggtcccgctcctgctccaggctctgccgcatctccgccatggtcagctctaagttgtgtttcatttcggagagctcttgctggtgcagccactggagcttctctatctcgatcctcagcctgcgaatctcagctattgtgcttccagtagtgtttttagaaagatcgttgtatatttctgtcattgttccttttattgcatccatcattttgctagtgtacttggcaatatcagcggcgacatcagctgaggcagtggcgatgggcaggtcagcgttgactgaggacacaagggtgctcatggaccccgagctggtgaccaggggcgatgactgtgtgctggtcaccagggtgatggtggacgtggatgggctctgtgtgatctccttctgctggacagttgatgagttccacacgacccgctgcacggccggggcagtctccttcggtaaaagcggcctctgctttttcactgggcttcctgtggcggcgggggccggggccgtgacggtgaccgtggaggacgtgctggtggtggctgtggcgccagccgcggaagtttgggcggaagagcgggtgagcaccggtgtttccgggggagaatggctgcccaccgtcgtggatggtggagttttacctacaacatcctgtttgggagatggttctttgggttccttcttattttttcgaccctcccgcccagaatggtcttctcctaaatctatgacaagttcgctctctgaatcagagtccaggcccaaatggactgttggggaatccgtctcatcttttcccttcagtttatcctttatggggtgaggtgaaggttttgccttttcggaaaagtccttctcaggctcagggctggccttgtccttgactgctccagggtctgccttctcgctggctggtgacgtgcttttcagctcctctttaatctccactgggtttgtaggcttgggcttttttttaacagcagatggctctttgtccatctgacaaccttctttgtcctctgtgtcttctggctcgttcttagacttctgctcatcatcactgatatactcactatcgctactatctgacttctcagaatcctccgaatcgctgtgctctacggccgtatagacatcttccgagatttcatttatgcctaattgtgctttgcaactctctatggtcttgtcaagattcagctggaacctgctacgaatctggcgcttgggagagatgagaggaacaggggtggactgttgctggaccgactcgctcagctccttcaaatccatctcagctttgcttcgatctgtgctcttatccaggaagtccatggactcctcgctcgcactgaagtggctcgacgtggccttcttctcagcatcctgctccacgtcggagcccgtgtgcacagaagagtttgtgctcatgggggagcgcggcatatccgacaaggaaatccggcggcctgtgcccccactcagcacaggcttgctcatcaggatcttgggggatgccgtcatgtcaaagttgagcttgaccttctcctgcttgtctatcttggcagtgccggcgctggggttggtgggatcgagcagcatttgatactggctgttgggtgtgtagggtgtcctaaatggagagtaattaaaaaccccaaacttcctgcggatgttctccacgtaaacctccatctcttgcatggcactgttgaagatgctcttagtctttttcacagaaaaaggaatttctttagacatgaggtagcaattatttattggaacccaggccctgtcatgttgtccaaagaatcgggcatcgacctgcccgtctttatcccttagagcttttgcaggccagaatggaaaccccttcagtttggcccagaccaaaggatgtggattgctacaaggctcacaaaaccagttatctcgtttttggcaagcagctagataacattctggacatacttcgatttcattcatctcatgttcacagattttgatgactactttcgctatttgcgtcaatttgtgatttcccccattataaatgatgcagttgtgcaaaatccactttgcatcagccaggaaggcttctgtgcagccatacattttctttttcgcattcttttccaatgtacaaaggtccattggatggaagatgtattccgcatagtcagggtgctgttccaatggaacgggcttctggaatgcatctgtccctggctgtttcattttctgaatggcaaacttgagcaggtaggataactgttcaatggtgagcattgtcatggctttactctgggtctcgatgcattctgctactgtaattttctcacattcaggacaaaaccagtccccctctggttccgatgtcagtctcagacacttagcgtgataaacccggggacagagctcacagcaaaggacttggccttcccggtgacaaacccagcagtagaaatcattccgtccatcctgctccttattgttactgttcagtaagccaggtttctttttctttttaatggggcttgttgatgtgtcctgcggcgagtggccattggaagaatgtggagggctggggaactttcttttctgggctgttctctctgcagagccaggatctttggagcgagtagagatatccatgccctctaccacctcctgttctgtttttatttcctcttcagccaagctctgtggatgcattgttaacactgtgtaatgtcaatacttat

SEQ ID NO: 18778 - RNA, 1442 nt, Homo sapiens
  source 1..1442: mol_type = other RNA
tgagttggccatctgagtgaggaccgaggtggccacagcttcagctgcagagcgaacactgaggccattgctaggggctgttgctgagctgtgctgaatcacaggggctggagaacccgttggctctgagctttccttggggctttctaaatagccttgagtctttttctgtagtgcagtgactgggcagtctttatgagctaacagtagctgtttcaactgggccacctcattgcgtagtaatgtgacttcattactcagctgaatgttctgagaagtgagttcttcggccttcttctctagggaggacacccacagctttcgcttttggcggcagcgggaggctgcagcccggttgcgctccagaaagcgctgccgtcgctcatctggatcttcatctactgtgcgccgccgtcgccccccagtactaggggtgggctgagctggtgagacctgtggctgggcaggggatggggcatcagggtgctggatgagaatctggctctgctctgggcgggctgtcaccatggtgctggcagtacccaccaccattccacaaccaccattgattgaggagacttggtgagttagggtggctttcagtctcatcttggcttctgatggtatagggtggccagagggagaaatggagccactactgttaactggtgggccagggataccaggaatgttgggcaccatggacacaggtctggccagcgatataacagacggcatctgtactggaggccctggcaacacaggcatggtctgtccattagcaagatgcatgacaagagggagggagccagtgggagaccccatttgcctgttggatggtggagcctgtgtgatgacagaggttggggagggaagggttggatgaagtggatcatagcccaagtggagaggcagggagccaggacgtacaatggtgggtgtgggggtagagatcagaacaggctttggggtaacctcctccactggctcttcttctttgattttgatgtctggtgtggaaggcagagacatgtcaaggggcccagcagcagcctttttctcatcctcatctgcagctttcttgaattcatgttcaaaggagctagctagttcattgaagagtcccacctcctcacagttcttcaggaatctagttggagtaggcgtttgatctgcaatgatgactgagtcagttcgggctgggccaaatttcaatgtcatctcatgcttgtgtttatgaactgccaggtggtcctcgtttgtaaatctctgtccacagcccggggcattgcacacaaacggtctgtcgtctcccatatttcatatagcagagaggagcggctggtagctccgttgcctcccgcctgcccgcgctcggtcctacaatctgtctccagctcctcctttccccccttggcggaacggatactttcctcccgtcc

SEQ ID NO: 18779 - RNA, 1538 nt, Homo sapiens
  source 1..1538: mol_type = other RNA
tgagttggccatctgagtgaggaccgaggtggccacagcttcagctgcagagcgaacactgaggccattgctaggggctgttgctgagctgtgctgaatcacaggggctggagaacccgttggctctgagctttccttggggctttctaaatagccttgagtctttttctgtagtgcagtgactgggcagtctttatgagctaacagtagctgtttcaactgggccacctcattgcgtagtaatgtgacttcattactcagctgaatgttctgagaagtgagttcttcggccttcttctctagggaggacacccacagctttcgcttttggcggcagcgggaggctgcagcccggttgcgctccagaaagcgctgccgtcgctcatctggatcttcatctactgtgcgccgccgtcgccccccagtactaggggtgggctgagctggtgagacctgtggctgggcaggggatggggcatcagggtgctggatgagaatctggctctgctctgggcgggctgtcaccatggtgctggcagtacccaccaccattccacaaccaccattgattgaggagacttggtgagttagggtggctttcagtctcatcttggcttctgatggtatagggtggccagagggagaaatggagccactactgttaactggtgggccagggataccaggaatgttgggcaccatggacacaggtctggccagcgatataacagacggcatctgtactggaggccctggcaacacaggcatggtctgtccattagcaagatgcatgacaagagggagggagccagtgggagaccccatttgcctgttggatggtggagcctgtgtgatgacagaggttggggagggaagggttggatgaagtggatcatagcccaagtggagaggcagggagccaggacgtacaatggtgggtgtgggggtagagatcagaacaggctttggggtaacctccttctccttcagtggtggggaacagggactagaggcagggctatcaggtggggatgagtctacctccactggctcttcttctttgattttgatgtctggtgtggaaggcagagacatgtcaaggggcccagcagcagccaccagttttttggcaacagtcctgcttcttgcctttttctcatcctcatctgcagctttcttgaattcatgttcaaaggagctagctagttcattgaagagtcccacctcctcacagttcttcaggaatctagttggagtaggcgtttgatctgcaatgatgactgagtcagttcgggctgggccaaatttcaatgtcatctcatgcttgtgtttatgaactgccaggtggtcctcgtttgtaaatctctgtccacagcccggggcattgcacacaaacggtctgtcgtctcccatatttcatatagcagagaggagcggctggtagctccgttgcctcccgcctgcccgcgctcggtcctacaatctgtctccagctcctcctttccccccttggcggaacggatactttcctcccgtcc

SEQ ID NO: 18780 - RNA, 1333 nt, Homo sapiens
  source 1..1333: mol_type = other RNA
tgagttggccatctgagtgaggaccgaggtggccacagcttcagctgcagagcgaacactgaggccattgctaggggctgttgctgagctgtgctgaatcacaggggctggagaacccgttggctctgagctttccttggggctttctaaatagccttgagtctttttctgtagtgcagtgactgggcagtctttatgagctaacagtagctgtttcaactgggccacctcattgcgtagtaatgtgacttcattactcagctgaatgttctgagaagtgagttcttcggccttcttctctagggaggacacccacagctttcgcttttggcggcagcgggaggctgcagcccggttgcgctccagaaagcgctgccgtcgctcatctggatcttcatctactgtgcgccgccgtcgccccccagtactaggggtgggctgagctggtgagacctgtggctgggcaggggatggggcatcagggtgctggatgagaatctggctctgctctgggcgggctgtcaccatggtgctggcagtacccaccaccattccacaaccaccattgattgaggagacttggtgagttagggtggctttcagtctcatcttggcttctgatggtatagggtggccagagggagaaatggagccactactgttaactggtgggccagggataccaggaatgttgggcaccatggacacaggtctggccagcgatataacagacggcatctgtactggaggccctggcaacacaggcatggtctgtccattagcaagatgcatgacaagagggagggagccagtgggagaccccatttgcctgttggatggtggagcctgtgtgatgacagaggttggggagggaagggttggatgaagtggatcatagcccaagtggagaggcagggagccaggacgtacaatggtgggtgtgggggtagagatcagaacaggctttggggtaacctccttctccttcagtggtggggaacagggactagaggcagggctatcaggtggggatgagtctacctccactggctcttcttctttgattttgatgtctggtgtggaaggcagagacatgtcaaggggcccagcagcagcctcctcacagttcttcaggaatctagttggagtaggcgtttgatctgtccacagcccggggcattgcacacaaacggtctgtcgtctcccatatttcatatagcagagaggagcggctggtagctccgttgcctcccgcctgcccgcgctcggtcctacaatctgtctccagctcctcctttccccccttggcggaacggatactttcctcccgtcc

SEQ ID NO: 18781 - RNA, 1441 nt, Homo sapiens
  source 1..1441: mol_type = other RNA
tgagttggccatctgagtgaggaccgaggtggccacagcttcagctgcagagcgaacactgaggccattgctaggggctgttgctgagctgtgctgaatcacaggggctggagaacccgttggctctgagctttccttggggctttctaaatagccttgagtctttttctgtagtgcagtgactgggcagtctttatgagctaacagtagctgtttcaactgggccacctcattgcgtagtaatgtgacttcattactcagctgaatgttctgagaagtgagttcttcggccttcttctctagggaggacacccacagctttcgcttttggcggcagcgggaggctgcagcccggttgcgctccagaaagcgctgccgtcgctcatctggatcttcatctactgtgcgccgccgtcgccccccagtactaggggtgggctgagctggtgagacctgtggctgggcaggggatggggcatcagggtgctggatgagaatctggctctgctctgggcgggctgtcaccatggtgctggcagtacccaccaccattccacaaccaccattgattgaggagacttggtgagttagggtggctttcagtctcatcttggcttctgatggtatagggtggccagagggagaaatggagccactactgttaactggtgggccagggataccaggaatgttgggcaccatggacacaggtctggccagcgatataacagacggcatctgtactggaggccctggcaacacaggcatggtctgtccattagcaagatgcatgacaagagggagggagccagtgggagaccccatttgcctgttggatggtggagcctgtgtgatgacagaggttggggagggaagggttggatgaagtggatcatagcccaagtggagaggcagggagccaggacgtacaatggtgggtgtgggggtagagatcagaacaggctttggggtaacctccttctccttcagtggtggggaacagggactagaggcagggctatcaggtggggatgagtctacctccactggctcttcttctttgattttgatgtctggtgtggaaggcagagacatgtcaaggggcccagcagcagcctttttctcatcctcatctgcagctttcttgaattcatgttcaaaggagctagctagttcattgaagagtcccacctcctcacagttcttcaggaatctagttggagtaggcgtttgatctgcaatgatgactgagtcagttcgggctgggccaaatttcaatgtcatctcatgcttgtgtttatgaactgccaggtggtcctcgtttgtaaatctctgtccacagcccggggcattgcacacaaacggtctgtcgtctcccatatttcatatagcagagaggagaccaagttctccccacacttcaagcctctggccccgcctt

SEQ ID NO: 18782 - RNA, 1505 nt, Homo sapiens
  source 1..1505: mol_type = other RNA
tgagttggccatctgagtgaggaccgaggtggccacagcttcagctgcagagcgaacactgaggccattgctaggggctgttgctgagctgtgctgaatcacaggggctggagaacccgttggctctgagctttccttggggctttctaaatagccttgagtctttttctgtagtgcagtgactgggcagtctttatgagctaacagtagctgtttcaactgggccacctcattgcgtagtaatgtgacttcattactcagctgaatgttctgagaagtgagttcttcggccttcttctctagggaggacacccacagctttcgcttttggcggcagcgggaggctgcagcccggttgcgctccagaaagcgctgccgtcgctcatctggatcttcatctactgtgcgccgccgtcgccccccagtactaggggtgggctgagctggtgagacctgtggctgggcaggggatggggcatcagggtgctggatgagaatctggctctgctctgggcgggctgtcaccatggtgctggcagtacccaccaccattccacaaccaccattgattgaggagacttggtgagttagggtggctttcagtctcatcttggcttctgatggtatagggtggccagagggagaaatggagccactactgttaactggtgggccagggataccaggaatgttgggcaccatggacacaggtctggccagcgatataacagacggcatctgtactggaggccctggcaacacaggcatggtctgtccattagcaagatgcatgacaagagggagggagccagtgggagaccccatttgcctgttggatggtggagcctgtgtgatgacagaggttggggagggaagggttggatgaagtggatcatagcccaagtggagaggcagggagccaggacgtacaatggtgggtgtgggggtagagatcagaacaggctttggggtaacctccttctccttcagtggtggggaacagggactagaggcagggctatcaggtggggatgagtctacctccactggctcttcttctttgattttgatgtctggtgtggaaggcagagacatgtcaaggggcccagcagcagcctttttctcatcctcatctgcagctttcttgaattcatgttcaaaggagctagctagttcattgaagagtcccacctcctcacagttcttcaggaatctagttggagtaggcgtttgatctgcaatgatgactgagtcagttcgggctgggccaaatttcaatgtcatctcatgcttgtgtttatgaactgccaggtggtcctcgtttgtaaatctctgtccacagcccggggcattgcacacaaacggtctgtcgtctcccatatttcatatagcagagaggagcggctggtagctccgttgcctcccgcctgcccgcgctcggtcctacaatctgtctccagctcctcctttccccccttggcggaacggatactttcctcccgtcc

SEQ ID NO: 18783 - RNA, 2746 nt, Homo sapiens
  source 1..2746: mol_type = other RNA
tgagttggccatctgagtgaggaccgaggtggccacagcttcagctgcagagcgaacactgaggccattgctaggggctgttgctgagctgtgctgaatcacaggggctggagaacccgttggctctgagctttccttggggctttctaaatagccttgagtctttttctgtagtgcagtgactgggcagtctttatgagctaacagtagctgtttcaactgggccacctcattgcgtagtaatgtgacttcattactcagctgaatgttctgagaagtgagttcttcggccttcttctctagggaggacacccacagctttcgcttttggcggcagcgggaggctgcagcccggttgcgctccagaaagcgctgccgtcgctcatctggatcttcatctactgtgcgccgccgtcgccccccagtactaggggtgggctgagctggtgagacctgtggctgggcaggggatggggcatcagggtgctggatgagaatctggctctgctctgggcgggctgtcaccatggtgctggcagtacccaccaccattccacaaccaccattgattgaggagacttggtgagttagggtggctttcagtctcatcttggcttctgatggtatagggtggccagagggagaaatggagccactactgttaactggtgggccagggataccaggaatgttgggcaccatggacacaggtctggccagcgatataacagacggcatctgtactggaggccctggcaacacaggcatggtctgtccattagcaagatgcatgacaagagggagggagccagtgggagaccccatttgcctgttggatggtggagcctgtgtgatgacagaggttggggagggaagggttggatgaagtggatcatagcccaagtggagaggcagggagccaggacgtacaatggtgggtgtgggggtagagatcagaacaggctttggggtaacctccttctccttcagtggtggggaacagggactagaggcagggctatcaggtggggatgagtctacctccactggctcttcttctttgattttgatgtctggtgtggaaggcagagacatgtcaaggggcccagcagcagcctttttctcatcctcatctgcagctttcttgaattcatgttcaaaggagctagctagttcattgaagagtcccacctcctcacagttcttcaggaatctagttggagtaggcgtttgatctgcaatgatgactgagtcagttcgggctgggccaaatttcaatgtcatctcatgcttgtgtttatgaactgccaggtggtcctcgtttgtaaatctctgtccacagcccggggcattgcacacaaacggtctgtcgtctcccatatttcatatagcagagaggagcttacaacttccatgtgtaagtacaaattgtgtttgatttccccagcccttggcctaagatattatgacatagctttagtttctgagtctggacacaaaggaaaaaactgaacatttttcactttcctgaaataacatgtctattttatttacactatttaaaaacacattatgtaagttaactaaaacaaactgcaaccacccattcgacaactcttcgagaatgactggggaagccacatttaacaaaacaaacttcattttagtatatttctgcttagaatgcccataaagactgatatcgctacaagaattacactactgcaaaatttttaaacacaggactcatgtgagcttgctgagaaaactctgcacaccccctacacacctgtacttaatatgacatgaccctcagagatactaaaacaccctctgttaagcagaaaacaaacttttaaagttaggaaagtagcaacgcgggaatctgggtaggaggtgccctgggttgtaaacaccccagtcagagaacataacaagcaattcagagcaacatattaagtccctatggggctccaacttggactgcttaagtcccaagaccacatcctggtgtctgggaagagtttgggtaatagaagagagggagaaggaaaatcagagaagcgatgaaagcgttctatttttctccttctcaacccccatcccagcatcttggaggctggtcaccagtctgggtgccatatccaccagaagccctaaatcaatatcccaaccacctgatacctaggctaaagacatgtgtatatcagccatctccttcccaaacacctcttatcgctctcaaggctcatatccttccagaagccatgccttatggcgactcagctcacccatactgtcctcttaaattaattcacttaattttctccaaatccatactttctctctgatatcatgtccctgatgttcttttaattaattcaatcaaaatgccatgaccctcatttccaataatccaccccatctatcttttctgccaaacccaacggggtgttgtgtcaccagatcaagatctttgttctcatctactcattcctacctccttcctattacccttttccaattccaagctcctaatcccactctttgggaagccctgggtttctaacttagtttagtatccctcctctttctcccattccaccccatcccatgatccttccattaggctccactagactacccttccctcaggattcaattcccctctccttgccacgccctgtgccccccggggctacttacaccaagttctccccacacttcaagcctctggccccgcctt

SEQ ID NO: 18784 - RNA, 4020 nt, Homo sapiens
  source 1..4020: mol_type = other RNA
tgagttggccatctgagtgaggcaagctttgagatgactgctgcaccagccattgactgcagcctcatgagagaccctgacagcgagcagcccggctgagcccagtcagctcccagacaccagaagagaaaacggccataaacgatgctacgccgctgaggtgggcggtttgtcatgcagctgtagatgactgatcttctccttgctgggcatgaccaggagcgaaggggatcccatcagtggaaatgcttcataaactgtaaagtgcagtgccgcaggtccatgtgtggcgtgctccctagatcaccactgcagtgaagtggaggactgggagtgttgagggagcggctgtgggggaaaggcctcccacgtcctgaggcccgagtcaggcttcctttcaaagccagccctgtttcccgtcctttccctgccttgatggggctgtcgggggcttttggtcattgccagggatggggccctcagcgtccacatgtctcagatttcatctctgccggcagccctagagtctgcgagtcgagatcatcatctataaactcctcaccctggacagcgccctggacgtcctcactgtgactcacagggctggtcatctcctgctccttctcgttgtgcatttgggcgtacacggtcctgcctggccgtttcctgcttttgaacttgtagaggatgaaggctcccgctgcgaagagcccgatgacaaacagcaccactaccgcccagtagccgccaccgccgcccagctgctcagcacctgtgcctgtgtcccgcagggccaccaggacccggactccgcctcgcaggaggaagctgatcttctgtgcgttcagcacctgctggatggcggcgagcctcttatcactcgagaggctcctcttccttgtgggcctgggagggggcaggagcacgtacagatcggccaaagtgggcagccccggcttcaccacagtcaccagaagctcctgagggacgctggtctccttggagagcagccgggtgaccaccaggcccacgtcttccctccactcaggggtgttggggttgtaggcatccagctccttggaaaactgcagaggcatgacttgaaattgatccagcacacggaggaccctggagtcctgcagcaccgagttcccacaggcggcctgcaccgtcacacgcacgtcgcccgtgtccgaaaaccgcgttgtcacagaattatccagggaaaggaggggctgcaggctgtggccgatccaccagtagaagacggtgaggttagggttcaagggaagcagcacagctgtgaggttcacctcctggttgaggccaatgacaggaaccacctccaggtagagggcctgcaggggggagttgacctggacaaagagcaccgcctcatcgtggcctgccgtgttctctgccctgacggacacgcggtagatgccggggctctcgtagcggtgccggatgggctccccggtcagtgtaaggttcacgtacatggccttgaagccgtccccaaggtctacctggtacttggtagtcaggacatcaccctgctcctgccgcaccacaaacaggacgtcctctccaggccgcacggccaccgcctcgccttgaatgctgacctgcaggccccggggcggcgtgagggggcactgcagctgcacctgactctgctgcatgtccaccccaccctcacacacgttggacaccactttccggtacccaaggctgctggtgtaggtctggcccagggcacagtcgtcaggcggggacaatgggttaaaccagaagttggcagagcacttgttggtgctggactctgaggaggaggagcgctcaaatccgtagtcgcacaggaagtccgagtcccggcactcgcacacgcgggacgtgagcgccgacgtgaagctcctccccttgatgcaccaggacgtggactttcttttccggaaacttctctgctggcccatgatacagcggtcgccctgcaggttggagagctcccaggagctgtagtcctcctcgccgcactgcctggagaatgagggccggaagtccaccttgaccagctcccaatcggagcggaagctgatgtggccaaagaccgtcatgaccagcgtctcgtcccctggctcactcagcagcccgtccacaaacaccgaggtgctggtgaagttgtgcgtgctccaggtgaggccctcgtccacactgaacttgaggatcttcaaagggatggaggtgtctttgatggccacgatcacgccgccgtggtccaggtacaggatgtgatgctcttcctcaaacacctgccgccaggtgtgaccacagtctgacgtgatgtacatttcttctttatattccaccagctgtgagcccaggttacctgcacccatgatgaggcctggggcggtgtccttggtgtgcacggtgcctgatacgtaggggttgtctgcccagcgcaggtgcaggtgcaggtggcagtctggaggcttgcagttggttggttttccattcatgtccatgctgggtggcctcaggtaatcccagtcgcggcccttgttgtaggttataagcgtcatcactttcccatcaattttttggtttgccaggaagactcctttcacccctctgacctccaggatgtcgatgagcacgctctcctccgcctgccgtgagctgcgcacgtcctgcagcaccagcgcgtagcgcacgccccgtgggtccgactggtacaggttgtaggtgtccatctggtaccactcctgcaccgccacgaacacctgactctcgtccgtgctgatgatctgcagatcctttggcaatgcatacttcggcagcttcatcaggacaaattcatttcgacgataagagacgtagtattttgtctggtttgctgatgttgccttaaagaagatgtaatcgtcctgcacggtcagagacccgtggtcaatggggcctgcgaatggggctgtcagcatcttctcggagcaattgtggattgcgcaggtgacgtaccgaaaatctccaccgaggtcttgggcttccacgtggaccaagtcagggtcagcgtccaccccagacacagaccagaacacgtggtctttggtcactcgctcttgcagaagtgtccactttttccccaagtcagatgacacgtagagcttgctctcctttgtgtaggcgaggaccttgtcctcctccttagggtggaaaatcagagtttccacgaagaagggaatgggctgcttctgaaaggtggcgccttcgtctgcgctgaggaataggctctggtcccggtcactgagtgaggagctgacaaggatgaccttcctcttgttggtcgggcagatgtagaaattgtcgatgacggtggtgacaccaggctggagggtgagcttggtgtaggacgtcccgaaatctgatgaccgccacagagaactttccagaaccttccccatgtctgcgtggtagtacttcgtcaggatcaagatcacgctgctgttctcgcccgtccagtgcaccatcgcctggttgtgcgtcgcgtcccccttgagcacgaacgacgtgctgatgagcgagacctgcgcccgcgaagccactccggccagcggcgccgcccgctcccagcgccggtagcccgcggcgggggcgccgtcctcgccgggaccaggagcgggaccgggactcggacccggggcgcctggctccgtgccgcgcgcctgccggtcctcgccgccaccgggctccgcgcgccccgcgggagggctccgcggcacccgggtcagttgggcgtgaggacccaggcgcccgggctcaggggagcgccccgccgccccgcaggcgcccagcagcagcagcagcagcaggagcggccgcgagcgcggcgagcgcggcggcggcggagccccggggctcggggctcgggcggtggggccggggcccttcgaggcgcgcgagggcccccggtgcgccatggtcgccaggggcggcagcggagccggcggcggggcggcg

SEQ ID NO: 18785 - RNA, 559 nt, Homo sapiens
  source 1..559: mol_type = other RNA
tgagttggccatctgagtgaggtcccgcttcatggcataggcgtcctccccatctgcatagtatttgggctccacttcactgatcctcttcctgacatgcagggagacatatttggcattgaagttctctatcatggctcgagaggcctggtccatcagtttctgagccagaccgaggcgccggtgggaacgcttcacagccaatgaggtgatatgtccatggggcacatcatctgggtcctcttccattttggccaggacataccccacaatcttcccattctcgtcctcagcaatgtaagagagctggggccaggaaaggccatggtagaagtagtatttcatctggtagttctcgggcaggcagaggaggttgcagtgctgcatgttcattaggtcctctggcctcgcattgcggatgttcataacggcggcggggctcgcgggtcccagcggatcgtgaaggcgcagtcagctgccgccgcgctccgaagcgacgccgggacggccggggctgggaccggagctgggctcgctgggcgacggcggaaggggcggt

SEQ ID NO: 18786 - RNA, 604 nt, Homo sapiens
  source 1..604: mol_type = other RNA
tgagttggccatctgagtgaggtcccgcttcatggcataggcgtcctccccatctgcatagtatttgggctccacttcactgatctgaaagttgagggtgttggaatagaggtgcagggcggcccggttactcttcctgacatgcagggagacatatttggcattgaagttctctatcatggctcgagaggcctggtccatcagtttctgagccagaccgaggcgccggtgggaacgcttcacagccaatgaggtgatatgtccatggggcacatcatctgggtcctcttccattttggccaggacataccccacaatcttcccattctcgtcctcagcaatgtaagagagctggggccaggaaaggccatggtagaagtagtatttcatctggtagttctcgggcaggcagaggaggttgcagtgctgcatgttcattaggtcctctggcctcgcattgcggatgttcataacggcggcggggctcgcgggtcccagcggatcgtgaaggcgcagtcagctgccgccgcgctccgaagcgacgccgggacggccggggctgggaccggagctgggctcgctgggcgacggcggaaggggcggt

SEQ ID NO: 18787 - RNA, 586 nt, Homo sapiens
  source 1..586: mol_type = other RNA
tgagttggccatctgagtgaggtcccgcttcatggcataggcgtcctccccatctgcatagtatttgggctccacttcactgatctgaaagttgagggtgttggaatagaggtgcagggcggcccggttactcttcctgacatgcagggagacatatttggcattgaagttctctatcatggctcgagaggcctggtccatcagtttctgagccagaccgaggcgccggtgggaacgcttcacagccaatgaggtgatatgtccatggggcacatcatctgggtcctcttcccccacaatcttcccattctcgtcctcagcaatgtaagagagctggggccaggaaaggccatggtagaagtagtatttcatctggtagttctcgggcaggcagaggaggttgcagtgctgcatgttcattaggtcctctggcctcgcattgcggatgttcataacggcggcggggctcgcgggtcccagcggatcgtgaaggcgcagtcagctgccgccgcgctccgaagcgacgccgggacggccggggctgggaccggagctgggctcgctgggcgacggcggaaggggcggt

SEQ ID NO: 18788 - RNA, 12254 nt, Homo sapiens
  source 1..12254: mol_type = other RNA
tgatatgtttgatattgggttgtctttttgttgttgggttgtaagagttctttatatgttctggatactagacccttatcaggtatattattttacagtgtcttttctcctatattcaccttttttttttttgagacggagtctcgctctgtcgcccaggctggagtgcagtggtgagatctgggctcactggttccaggttcacgccattctccttcctcagcctcccaagtagctgggactacaggcttccactaccagcctggctaattttttgtatttttttgtagagacagggtttcaccacattagccaggatggtttcgatctcctgacctcgtgatccacctgcctcagcctcccaaagtgctaggattacaggcgtgagccaccacacccggccttttttttttttttgagatggaattttgctttcttgctctgtcacctgggctggagtgcagtagcatgatctcggctcactgcaacctccacctcacagcttcaagcgatcctcctgcctcagcttcctgagttgctgggattacaggcacatgccaccacacccggcttttttttttctctttttttttatttttagtagagacgtggtttcaccaagttaaccaggctggtctcgcactcctgacctcaagtgatcctcccaccttggcctcccaaagtgctggaattacaggcgtgagccaccacacccagctccttttcactttcttgatagtgtccactgatgccgaaagttttcaattttggtgaagtccaatttacctattttttcttttgtttcccatgcttctggtgtcatatccaataaatcattgccaaatccagtgccaagaagtacatgaaaagattttcaacatcactagccattaggtaaaggaaaatcaaaaccacaatgagataccatttcatacatgttagagtggctattataaaaaatatggaggccaagtgcagtggttcaagcctgtaatcccagcactttgggaggccaaggtaagtggatcacttgaggacaggagtttgagactagcctggcctggccaacatggtgaaaccctgtctctactaaaaatacaaaaaatagccatacatggtggcacatgcctgtaatcccagctactcaggaggccgaggaaggagaatcacttaaacctaggaggcggaggttgcagtgagctgaaatggtgccactgcactccagcctgggtgacagagtgaaactccatttcaaaaaaaccaaaaaactatttgggtgtagtggcacctgtagttccagctacccaggaggctgaggtggaaggatcccttgagcccaggaggttggggctgcagtgagttatgatcatgcctatgaaatgagagagaaacaaactaattaatattggcaagtatgtggagaaattggaagccttgtgcactgctggtggaatgtaaaatgatagttgcacaataatggaaataatgtacttcatgccactgaagtgtacacttaaaaatagttaaaatggtaaatgttcttattatatatatgtgtatatatatgtgtatatgtgtatatatatgtgtatatatgtgtgtatgtgtgtgtgtatatatacatatatatatatatatatatatatatatatatatatatatatatatatatataaaatcacacatgaaagtctcccttggaactgatcctgaaataatttcatgtgtgatgaaagaacaccctgctctcctggagtgataagtggcctttttgttcatgctggcattatacatcccaggctcttccacacacacccagcataatttcaccaagcagagggagtacactctccaaaggcccatttgtgcctgtttctatcattatatcctcctatttaactcactccctgccctctacaaaccgtcatcaatcacagatatgtttgctacccctgtagtttctgcttttccataacatcatagaaataggatcatacagccttttcacactggtctctttcacttagcaatatgcctatcagattcatccatgtcctgcatggcctcagagcttgctcttgctgaacaggactccattgcatggatgtaccccagcctagttagtcattcacctattgaaggttatcctgattccttaaagtatttgtctgttatgaaaagagctgctgtacgtgagtacatgctgggttttgtttagatcaaactcctatgttttcaaagcagttatctaaatacctaggagtgtgattgttggctcatattgtgaagctttgtttagctttggggaaaagtcaaactatcttccaaagtggctatactattatgcattgcaccagcaatgaatgagagttcctgttgcaattgcaaatttacttatttttagattatagtcactttaatagatgtgcggtgctatctcgttgttttaatttgcttttccctcatgacaagtgtcactgagcattatttggtatgcttatttgccatctgtatatcttcttttttttttttttgagacggagtttcactcttgttgcccaggctggagtgcaatggcgcgatctcggctcacagcaacctccgcctcccgggttcaagccattctcctgcctccgcctccggagtagctaccacttggtggcagagtagcgccaccacgcctggctaattttgtatttttagtagagacagggtttctccatgttggtcaggctggtctcgaactccggacctcaggtgatctgcccgcctcggcctcccaaagtgctgggattacaggcgtgagccaccgtgcctggccaccatctgtatatctttggaaagtatgtatttggatctgtccccatttttaattgggttgtcttcttgttcaattttagggttttttttttatattttgcatacaaacactttttcagatttttttgaatgattttattcattacaaattccaattattgctatacattatttcaaatatataggaaatcacttgacttttgtctatggccatctactttgccttttattatctctatccattccaattaaggcatggaatgatggactctatttcagtttcgttttccaaaattatggcatggaaaatcgtaagattgaatttcaggggttcactgggactgcaagagggggcacatggccatcacaaaacaggaagcactgaccatccaacactgtgcctaggtagtaaggaaggggtgcaagcacacaccttgtctagcctgcttgcagtacctgcattctgctcacagacctctgggttgaatccacagaggaccaggccttccttctactcaggacctggggatcactagaggctgcatcacagtaaagactgagctgccttctcctcaggactgacctggggacccttggcaggggggaatccacagtgacaaacagaccttgcttctactcaggacccggagacccccgagggcacttcacagtgatgaccagaatttacctcatctcaggaccaacctgggggatgcatcacactgagaaccagagcttccttctccactggccaacctgaggaccactgtggggcacaaccacagtgaagactggagcttgtttctcttcaggactgacctagggaccctagtggggcaaatccacagtgaggttctgagcttccttctcctcaggaccaacctggggacccctgggaggtagatcacagtgatgaccagagtatcctcctcaggactgacccgtggtgggggatgcaaccacagtgaggactaaagcttccttttcctcacaacctggggaccccctagggggatacatcacagtgagatccagagcttccatatctgaagactcctgtagggtacacccacagtgacgaccagtgcactttccggaccaatctggggcgatgtcatctcacctttgggatacatggaggccacaggaggaaaagatgaggaaaagtgaggcctgcaccctgagtgctgaggagggagctttgctgtttcactttgccctgtaatatctgaacaagatttattttaggaaatcgtacctctattgaggtttccactagtcatctttatagcaagcccaactactttttatacatatgggtttgtttctggggagaaatcccagtacaaaaaaagggagaaacactgcgacaaaacactgcaacagtccaggtcaaagttggggatgaacagcacctgtgggatcaccctggatcccaagagggaagggcaaatgtgcaccctatgtgcttgcttttattaattttttttgaaggagtctcactctgctgcccgggctggagtgcaatggcacaatctcagctcactgcaacctccgcctctccagttcaagcaattctcctgagtagcttggattatagatgcatgccaccacagctggccaatttttgtatttttagtagagacggggtttcaccaggctggtctcgaactcctgacctcaagtcatccacctgcctcagcctcacaaaatgctgagattacaggcatgagccaccatgcccagcctttttattaatgttttaatggcctgtgtttctaacaagtagttgaaacaatgttgaaaattaaagagtagacatgttaaaacttgcaacttcatttaaatttaaatatatcatttataccaaaatcagaatttatttaagatttatggctgggtgcttggctcacacctgtaatcctagcactttgggaggccaaggcaggtggactgcttgagcccaggagtttgaaaccagactggaaaacatggtaaaaccccatctctacaagaaataaataactctacctggccctttagcaaagaattaagaaaaatcaatacagaccagtggctcacacctgtaatcccagcactttgggaggctgagggtggatcacgaggtcaggagttcaagaccagcctggccaacatggtgaaaccccatctctactaaaaacacaaaaattagctgggcgtggtggcgtgtgcctgtaattccagctactagggaggctgaggcaggagaattgcttgaacccaggaggcagaggttgcagtgagccaagaacacaccactgcactccagcctggcaatacagcgagactccatctcaaaaaaaaaaaaaaaaatgcaaatactatgccatataaggagcttgagcatccacagggagtatctgtggttgcgggggggtcctccatgaatactgacaactgcatacttgctactctactggcagttccaaacatttgtttgtggtttattttgggtttcctaattacacgatcacatctccaattcatggcagttgtttctgcacccatccctaattcctcacattccttgttttcacaccttggctagatgttactcatttcataaaagtgatgcgcattcttgtaattttgctttgttttttacagacagggtctcactttgttgcccaggatggagtgcaggggcatgatcatagctcactgtagccttgaactactggactcaagctaacctcctgcctcagcctcctcagtaggtgggactaccggcacttgccactacacctggctgatcttttttttgagatggaggcttgttctgtcgcccagcctggagtgcagtggtgcaatcttggctcactgcaactgccacctcctaggttcaagcaattcttctgcctcagcctcccgagtagatgggattacaggcacgtgccaccacacctggctgacttttgtatttttagtagagacggggtttcaccatgttagccacactggtcttgaaatcctgacctcaagtgatctgcccacctcggcctcccaaagtgctgggattacaggcatgagccacggcgcctgaccacacctggctaatctttttaaaaagtttttgtacagacagggtctccctatattggtcaggcttgtctcgaactcctgggttccagcaatcctccagcctcagccttcccaagtgctggtattacatggatgagccactgcacctggctaattttactttaaaggaatctttctactattttatcattaagtatgacatttgtgttttcagaacatatattccctaccaagttacaggagttaattttaattcccaacttaatagtattttagtgtcatctatgggtgttaaattccatcaagtgatttatcagcatatactgagataatccttatgagttttatctggtagttaattaaaatattttctaatattaaatcttccaaacatactcttctgttttttgagacagggtctagttctgtcacccagggtggagtacagtggtacgatctcagctcactgcaacttccgcctcctagattcaagtgattctcccgtcccagcctcccaagtagctgggattataggtgtcagttaccatgccctgctatttttttgtatttttagtagagaggggtttcaccatgttggccaggctggtctcaaactcctgacctcaggtgatccaccatctcagcctcctgaagtgctgggattataggtgtgagccaccgtgcctggccccatatatctctttttaagtgggcatactgccattataaataatagtgattctgctggtaatgaacaaaggatgctggatccactaatagtctgttaaacctaatatcatgactttcttgttagctatacattggtttgctataattccatttagaatttttaaacctatgttcacaaatatggatttttaaacctatgttcacaaatatggatttttaaacctatgttcacaaatatggtttgcaagtcattttttctcctaaatttctatttgatggggaagttgtaaaatattggggttatttttccttggattttccttataataactattcctgaaaagtctctggaatgtctttcttttctggggctggggtagaaggactagatagatttacaaaccagtaactcaatttctgttttgtaaaattttcatttcattaaataataagtcctaatcaagtattattctttcccacagtatgtgagtgctgtcctcaatactgtcaacacttctggcttctaccaggcaaggctgcatgtagatttgcatctgaaaaaacaacaaactaaaatctaaccctaggtagtagtaaactgaatataaactttctcttatgaatttattctgtcttctttggtacatcaataataatatacacctttacagtatttcccagattgggggatacactttagcaagtatctgcgattatttgtttatgtaagatgtcccttcccttctgtgaatcatcattcttcaccccaagtatcttgagattggattctgtataagcagaatacaacagttaggcattcaggtatcattaaattcctccgcttcaaggatgaaaatttctttgggtatctaatagagtacaaagcagaaggtgtttcagaaatatttgcagtattgaatccgcatattcctccaagatagccctaatctaactggcagggtcccactcttcccagattaatgcccactcacataacaaacctgatgaggtagtgaagaaaactaactttgtgagtaagcaactggcagagtttttcaccactgtgactctatagctacatgtaactaagtagtatcactgacacataatcttaaattgaagttttaagatcattattctccatgttatacatgggtatcaaaagcattcccctcttgaccactccagaattctgtttaaaatttttcaatgacaacttatccatttccccaaagcctcagtgagcacatgatgccaacaattcatttcatgacttcatagcatgggccaagtttcttgcttaaaagacttccatcctgtcttgggaaacaaccatttccaaatatccacatatccttgcaagtttctgcctactcctctaccacccatttctgaagccatctgatttagtaagctgtatgcaaaagatacacaatggctaatgcaatcaaacaaggaatgtattaaaagcacacccaatagctcaaaataaaagacaagtgaacaaagttaagaaaatgacagtaacaaaagctgttctgggaacctctattgaaatagctacttattacatcaacatgctaccacagaacaaaagctcatgttgcttttctgaacttgaaaaacccattaacaatgtacagttctgagcctcagctgaccatagtgctcatgccaagtcctgagcagggcatcttgaatggtggttccctcatgactacatacaccgttagggaatgtttcgttaagaggaaatcaagatgttctaacctgtgaaggtagaatagattccaggctacacaaacacatgaagtgtgccttatattgattactaaagaggttgctgccaagactgcttccaaagggcagaagatagccctaaaaaatgtttgcagtgtggaaatgcatttttagtaagtcatattctagtaacaagttgcatttggtaagacacaaagaaacaatgttggtatgcagagtagaaatctctggaagatgatattgtcatatcagagatattgtcagtatcagagatactgaaatctctggaagatgatttttgtctcacatatggcattcgcaagtaaaatgccaaactgcaaaattcatattatgtagtacacataggaagatatctaaatatccctgtaggctctgggatgttatttcttattcttaacctccttactagattcacttgtacaatgaaataatctgtatcttattatttataattgagaattttctcaaaccttttcctgaaattttggaacacctggaataaaatttcttaaaatgattcctaaaagaaataattcttcaaaattaatattaagatataataacaggttggtttttttttttttttttttttttttttttagaatgaagcttctaaggtgaggttaacagtccagctgtggtttatttggtacattcataagatgttcactcctatatatattttttccctaggggtttctcatttctagatttacactttcccttatagcatggtccctccaaggtatatgcttccgatacataaaatgtttgtaattttgttaattctgccattcattagctcaataatttctctcattaaaattctgtaaactatgaatttcaaagaagtctattctatattcatctggttcatgaagtttcctctttgtgaatcttattttagtaaaatgactttacaacgtttaacatggttcctcacctgtatgaactttttaaaaaaaggtatgacttgctgctaaaaattttcagagtggttactaaattcagttttcctgtgtattgtctactatctttttgcatgtaaagaacagctttctgtggatgcctttccatatgctgtgcattcataaagtttctattcagtatgagttttctggaagatgacaagatgattccacttacagagtttctctttatatatgattgtttctatctcttgtgaatccacttttcagagtttcgtaaaattatcaatgtttgtcatctacatgagttctctgatgcataatgagctgtgacttccaacaaaaggctttcccacattcagtgcacttacaaggcttctctcctgtatgtgttctctgatgtgcactgagaattgatttttgagagaaggttttcccacattcattgcacccatagggtttctctcctgaatgagttctttgatgtacaatgagttgagaattcctaatgaaggcttttccacactcactgcattcatatggtttctctcttgtgtgcattctctggtgtacaagaaggcgtaatttcccactgaaggatttctcacattgactgcatttataagggttgacccctgcatgagttcgctcatgtacaatgagtagtgatttccaaatgaaggctttcccacattcattacattcatatggtttttcacctgaatgagttctcatgtgtataattaggtatgacttgctgctaaaagctttcccacattcactgcacccataaggcttttcccctgcatgagttcgctgatgtgaaatgagctggtctttcctattaaaggctttcccacattcactgcattcatagggattttctcctgtgtgaattctctgatgcacaatgagttgtgaattgaaactaaaggatttcccgcattccctgcactcatgtggtttctctcctgtatgagttctcatatgtataataaggtatgacttgctcctgaaggctttcccacactcactgcatccatatggttttactcctgtgtgacttctctgatgtacaatgagctgggacttcaaactaaaggtttttgcacattgactgcatccatagggttttactccagtgtgcactcctttatgtacaatgagctgtgatttgaacgtaaaggcttttccacattcattacaactatagggtttctctcctgtatgagttctctgatgtacaatcaggtttgactttgtattaaaggctttctgacactcactacattcaaatggtttctcccctgtatgagttctctggtgtataataagctgtgactttaaaccaaaagcctttccacagtcggtgcattcataaggcttctctcctgcatgagttctctggtgtgaaataagctggtatttccgactgaaggctttcccacattcatggcattcataggggttctctcctgtatgaatcctctgatgtataatgagctgtgatttaaaactgaaggctttcccacaattgttgcattcatggagtttttctcctgtatgagtccttgtatgtataataaggtatgacttgctcctgaaggctttgccacattcattgcatacataaggtttcattcctgtgtgacttctctgatgtacaatgagctgtgatttcaaactgaatcctttaccacactgaatacacccatagggctttactcctgtgtgaatcccctgatgtacaatgagctgtgacttgaatgtaaaggcttttccacaatcactacaaacataaggtttctcccctgtatgggttctctgatgtaccataaggtttgactttgtattaaaggctttctgacattcattgcattcatatggtttctctcctgtatgaattctttcatgtataatgagctgtgattttaaaccaaaagctttcccacattcattacacacatatggtttctgtcctgaatgagttttctggtgtgaaacaagctggtctttcctactgaagactttcccacattcacagcactcatagggattctcacctgtgtgaattctctgatgtataacaagctgtgaatggaaactgaatgttttcctgcattcactgcattcatgtagtttctctcctgtatgaattctctgatgtacaatgaggtatgatttactactgaagtctttcccacattcattacaaccatagggtttctcttcggcatgagtttgctgatgcactagaaggtatgacttgctgctgaaggctttctcacaacagctgcatccaaagggtttttcgcccatatacatttgttggcacataagttgcgatttcttattgacggtttttccagattcaatactttcacagtattttattccaataacagtttgctcatgtttagaatggaagaatgattttccatgtacctgaaacccattaggattatttctagcataatcactagtgaaatctatatatttcaaactctttccatgcgtgccacatttatgaggtttttgtcttgaaagatactttgtactaagaagacatagttttccaaatgtagtgcattcaaagctttttgccgtacttcccagcttgtctttattttcctgatgccaatccataagatcatcaattttccagactgtgtccaaatagaagctgtccggaccctggtggccatccctacggtcagttttgtgtgcctcgctggaagtgacaggacgcgagggatgctccggctcctccaaaccctgaaggggcagcagaatagagtccagggtactgcctccacctccagatctgcagccagaagggttcgcaaccactccagactcggctggcccgttgaccacgacgggcgatgaacgctatctgaggaacaaggatctcgccatcggcgcggaacaatggcggccgctacgtat

SEQ ID NO: 18789 - RNA, 12455 nt, Homo sapiens
  source 1..12455: mol_type = other RNA
tgatatgtttgatattgggttgtctttttgttgttgggttgtaagagttctttatatgttctggatactagacccttatcaggtatattattttacagtgtcttttctcctatattcaccttttttttttttgagacggagtctcgctctgtcgcccaggctggagtgcagtggtgagatctgggctcactggttccaggttcacgccattctccttcctcagcctcccaagtagctgggactacaggcttccactaccagcctggctaattttttgtatttttttgtagagacagggtttcaccacattagccaggatggtttcgatctcctgacctcgtgatccacctgcctcagcctcccaaagtgctaggattacaggcgtgagccaccacacccggccttttttttttttttgagatggaattttgctttcttgctctgtcacctgggctggagtgcagtagcatgatctcggctcactgcaacctccacctcacagcttcaagcgatcctcctgcctcagcttcctgagttgctgggattacaggcacatgccaccacacccggcttttttttttctctttttttttatttttagtagagacgtggtttcaccaagttaaccaggctggtctcgcactcctgacctcaagtgatcctcccaccttggcctcccaaagtgctggaattacaggcgtgagccaccacacccagctccttttcactttcttgatagtgtccactgatgccgaaagttttcaattttggtgaagtccaatttacctattttttcttttgtttcccatgcttctggtgtcatatccaataaatcattgccaaatccagtgccaagaagtacatgaaaagattttcaacatcactagccattaggtaaaggaaaatcaaaaccacaatgagataccatttcatacatgttagagtggctattataaaaaatatggaggccaagtgcagtggttcaagcctgtaatcccagcactttgggaggccaaggtaagtggatcacttgaggacaggagtttgagactagcctggcctggccaacatggtgaaaccctgtctctactaaaaatacaaaaaatagccatacatggtggcacatgcctgtaatcccagctactcaggaggccgaggaaggagaatcacttaaacctaggaggcggaggttgcagtgagctgaaatggtgccactgcactccagcctgggtgacagagtgaaactccatttcaaaaaaaccaaaaaactatttgggtgtagtggcacctgtagttccagctacccaggaggctgaggtggaaggatcccttgagcccaggaggttggggctgcagtgagttatgatcatgcctatgaaatgagagagaaacaaactaattaatattggcaagtatgtggagaaattggaagccttgtgcactgctggtggaatgtaaaatgatagttgcacaataatggaaataatgtacttcatgccactgaagtgtacacttaaaaatagttaaaatggtaaatgttcttattatatatatgtgtatatatatgtgtatatgtgtatatatatgtgtatatatgtgtgtatgtgtgtgtgtatatatacatatatatatatatatatatatatatatatatatatatatatatatatatataaaatcacacatgaaagtctcccttggaactgatcctgaaataatttcatgtgtgatgaaagaacaccctgctctcctggagtgataagtggcctttttgttcatgctggcattatacatcccaggctcttccacacacacccagcataatttcaccaagcagagggagtacactctccaaaggcccatttgtgcctgtttctatcattatatcctcctatttaactcactccctgccctctacaaaccgtcatcaatcacagatatgtttgctacccctgtagtttctgcttttccataacatcatagaaataggatcatacagccttttcacactggtctctttcacttagcaatatgcctatcagattcatccatgtcctgcatggcctcagagcttgctcttgctgaacaggactccattgcatggatgtaccccagcctagttagtcattcacctattgaaggttatcctgattccttaaagtatttgtctgttatgaaaagagctgctgtacgtgagtacatgctgggttttgtttagatcaaactcctatgttttcaaagcagttatctaaatacctaggagtgtgattgttggctcatattgtgaagctttgtttagctttggggaaaagtcaaactatcttccaaagtggctatactattatgcattgcaccagcaatgaatgagagttcctgttgcaattgcaaatttacttatttttagattatagtcactttaatagatgtgcggtgctatctcgttgttttaatttgcttttccctcatgacaagtgtcactgagcattatttggtatgcttatttgccatctgtatatcttcttttttttttttttgagacggagtttcactcttgttgcccaggctggagtgcaatggcgcgatctcggctcacagcaacctccgcctcccgggttcaagccattctcctgcctccgcctccggagtagctaccacttggtggcagagtagcgccaccacgcctggctaattttgtatttttagtagagacagggtttctccatgttggtcaggctggtctcgaactccggacctcaggtgatctgcccgcctcggcctcccaaagtgctgggattacaggcgtgagccaccgtgcctggccaccatctgtatatctttggaaagtatgtatttggatctgtccccatttttaattgggttgtcttcttgttcaattttagggttttttttttatattttgcatacaaacactttttcagatttttttgaatgattttattcattacaaattccaattattgctatacattatttcaaatatataggaaatcacttgacttttgtctatggccatctactttgccttttattatctctatccattccaattaaggcatggaatgatggactctatttcagtttcgttttccaaaattatggcatggaaaatcgtaagattgaatttcaggggttcactgggactgcaagagggggcacatggccatcacaaaacaggaagcactgaccatccaacactgtgcctaggtagtaaggaaggggtgcaagcacacaccttgtctagcctgcttgcagtacctgcattctgctcacagacctctgggttgaatccacagaggaccaggccttccttctactcaggacctggggatcactagaggctgcatcacagtaaagactgagctgccttctcctcaggactgacctggggacccttggcaggggggaatccacagtgacaaacagaccttgcttctactcaggacccggagacccccgagggcacttcacagtgatgaccagaatttacctcatctcaggaccaacctgggggatgcatcacactgagaaccagagcttccttctccactggccaacctgaggaccactgtggggcacaaccacagtgaagactggagcttgtttctcttcaggactgacctagggaccctagtggggcaaatccacagtgaggttctgagcttccttctcctcaggaccaacctggggacccctgggaggtagatcacagtgatgaccagagtatcctcctcaggactgacccgtggtgggggatgcaaccacagtgaggactaaagcttccttttcctcacaacctggggaccccctagggggatacatcacagtgagatccagagcttccatatctgaagactcctgtagggtacacccacagtgacgaccagtgcactttccggaccaatctggggcgatgtcatctcacctttgggatacatggaggccacaggaggaaaagatgaggaaaagtgaggcctgcaccctgagtgctgaggagggagctttgctgtttcactttgccctgtaatatctgaacaagatttattttaggaaatcgtacctctattgaggtttccactagtcatctttatagcaagcccaactactttttatacatatgggtttgtttctggggagaaatcccagtacaaaaaaagggagaaacactgcgacaaaacactgcaacagtccaggtcaaagttggggatgaacagcacctgtgggatcaccctggatcccaagagggaagggcaaatgtgcaccctatgtgcttgcttttattaattttttttgaaggagtctcactctgctgcccgggctggagtgcaatggcacaatctcagctcactgcaacctccgcctctccagttcaagcaattctcctgagtagcttggattatagatgcatgccaccacagctggccaatttttgtatttttagtagagacggggtttcaccaggctggtctcgaactcctgacctcaagtcatccacctgcctcagcctcacaaaatgctgagattacaggcatgagccaccatgcccagcctttttattaatgttttaatggcctgtgtttctaacaagtagttgaaacaatgttgaaaattaaagagtagacatgttaaaacttgcaacttcatttaaatttaaatatatcatttataccaaaatcagaatttatttaagatttatggctgggtgcttggctcacacctgtaatcctagcactttgggaggccaaggcaggtggactgcttgagcccaggagtttgaaaccagactggaaaacatggtaaaaccccatctctacaagaaataaataactctacctggccctttagcaaagaattaagaaaaatcaatacagaccagtggctcacacctgtaatcccagcactttgggaggctgagggtggatcacgaggtcaggagttcaagaccagcctggccaacatggtgaaaccccatctctactaaaaacacaaaaattagctgggcgtggtggcgtgtgcctgtaattccagctactagggaggctgaggcaggagaattgcttgaacccaggaggcagaggttgcagtgagccaagaacacaccactgcactccagcctggcaatacagcgagactccatctcaaaaaaaaaaaaaaaaatgcaaatactatgccatataaggagcttgagcatccacagggagtatctgtggttgcgggggggtcctccatgaatactgacaactgcatacttgctactctactggcagttccaaacatttgtttgtggtttattttgggtttcctaattacacgatcacatctccaattcatggcagttgtttctgcacccatccctaattcctcacattccttgttttcacaccttggctagatgttactcatttcataaaagtgatgcgcattcttgtaattttgctttgttttttacagacagggtctcactttgttgcccaggatggagtgcaggggcatgatcatagctcactgtagccttgaactactggactcaagctaacctcctgcctcagcctcctcagtaggtgggactaccggcacttgccactacacctggctgatcttttttttgagatggaggcttgttctgtcgcccagcctggagtgcagtggtgcaatcttggctcactgcaactgccacctcctaggttcaagcaattcttctgcctcagcctcccgagtagatgggattacaggcacgtgccaccacacctggctgacttttgtatttttagtagagacggggtttcaccatgttagccacactggtcttgaaatcctgacctcaagtgatctgcccacctcggcctcccaaagtgctgggattacaggcatgagccacggcgcctgaccacacctggctaatctttttaaaaagtttttgtacagacagggtctccctatattggtcaggcttgtctcgaactcctgggttccagcaatcctccagcctcagccttcccaagtgctggtattacatggatgagccactgcacctggctaattttactttaaaggaatctttctactattttatcattaagtatgacatttgtgttttcagaacatatattccctaccaagttacaggagttaattttaattcccaacttaatagtattttagtgtcatctatgggtgttaaattccatcaagtgatttatcagcatatactgagataatccttatgagttttatctggtagttaattaaaatattttctaatattaaatcttccaaacatactcttctgttttttgagacagggtctagttctgtcacccagggtggagtacagtggtacgatctcagctcactgcaacttccgcctcctagattcaagtgattctcccgtcccagcctcccaagtagctgggattataggtgtcagttaccatgccctgctatttttttgtatttttagtagagaggggtttcaccatgttggccaggctggtctcaaactcctgacctcaggtgatccaccatctcagcctcctgaagtgctgggattataggtgtgagccaccgtgcctggccccatatatctctttttaagtgggcatactgccattataaataatagtgattctgctggtaatgaacaaaggatgctggatccactaatagtctgttaaacctaatatcatgactttcttgttagctatacattggtttgctataattccatttagaatttttaaacctatgttcacaaatatggatttttaaacctatgttcacaaatatggatttttaaacctatgttcacaaatatggtttgcaagtcattttttctcctaaatttctatttgatggggaagttgtaaaatattggggttatttttccttggattttccttataataactattcctgaaaagtctctggaatgtctttcttttctggggctggggtagaaggactagatagatttacaaaccagtaactcaatttctgttttgtaaaattttcatttcattaaataataagtcctaatcaagtattattctttcccacagtatgtgagtgctgtcctcaatactgtcaacacttctggcttctaccaggcaaggctgcatgtagatttgcatctgaaaaaacaacaaactaaaatctaaccctaggtagtagtaaactgaatataaactttctcttatgaatttattctgtcttctttggtacatcaataataatatacacctttacagtatttcccagattgggggatacactttagcaagtatctgcgattatttgtttatgtaagatgtcccttcccttctgtgaatcatcattcttcaccccaagtatcttgagattggattctgtataagcagaatacaacagttaggcattcaggtatcattaaattcctccgcttcaaggatgaaaatttctttgggtatctaatagagtacaaagcagaaggtgtttcagaaatatttgcagtattgaatccgcatattcctccaagatagccctaatctaactggcagggtcccactcttcccagattaatgcccactcacataacaaacctgatgaggtagtgaagaaaactaactttgtgagtaagcaactggcagagtttttcaccactgtgactctatagctacatgtaactaagtagtatcactgacacataatcttaaattgaagttttaagatcattattctccatgttatacatgggtatcaaaagcattcccctcttgaccactccagaattctgtttaaaatttttcaatgacaacttatccatttccccaaagcctcagtgagcacatgatgccaacaattcatttcatgacttcatagcatgggccaagtttcttgcttaaaagacttccatcctgtcttgggaaacaaccatttccaaatatccacatatccttgcaagtttctgcctactcctctaccacccatttctgaagccatctgatttagtaagctgtatgcaaaagatacacaatggctaatgcaatcaaacaaggaatgtattaaaagcacacccaatagctcaaaataaaagacaagtgaacaaagttaagaaaatgacagtaacaaaagctgttctgggaacctctattgaaatagctacttattacatcaacatgctaccacagaacaaaagctcatgttgcttttctgaacttgaaaaacccattaacaatgtacagttctgagcctcagctgaccatagtgctcatgccaagtcctgagcagggcatcttgaatggtggttccctcatgactacatacaccgttagggaatgtttcgttaagaggaaatcaagatgttctaacctgtgaaggtagaatagattccaggctacacaaacacatgaagtgtgccttatattgattactaaagaggttgctgccaagactgcttccaaagggcagaagatagccctaaaaaatgtttgcagtgtggaaatgcatttttagtaagtcatattctagtaacaagttgcatttggtaagacacaaagaaacaatgttggtatgcagagtagaaatctctggaagatgatattgtcatatcagagatattgtcagtatcagagatactgaaatctctggaagatgatttttgtctcacatatggcattcgcaagtaaaatgccaaactgcaaaattcatattatgtagtacacataggaagatatctaaatatccctgtaggctctgggatgttatttcttattcttaacctccttactagattcacttgtacaatgaaataatctgtatcttattatttataattgagaattttctcaaaccttttcctgaaattttggaacacctggaataaaatttcttaaaatgattcctaaaagaaataattcttcaaaattaatattaagatataataacaggttggtttttttttttttttttttttttttttttagaatgaagcttctaaggtgaggttaacagtccagctgtggtttatttggtacattcataagatgttcactcctatatatattttttccctaggggtttctcatttctagatttacactttcccttatagcatggtccctccaaggtatatgcttccgatacataaaatgtttgtaattttgttaattctgccattcattagctcaataatttctctcattaaaattctgtaaactatgaatttcaaagaagtctattctatattcatctggttcatgaagtttcctctttgtgaatcttattttagtaaaatgactttacaacgtttaacatggttcctcacctgtatgaactttttaaaaaaaggtatgacttgctgctaaaaattttcagagtggttactaaattcagttttcctgtgtattgtctactatctttttgcatgtaaagaacagctttctgtggatgcctttccatatgctgtgcattcataaagtttctattcagtatgagttttctggaagatgacaagatgattccacttacagagtttctctttatatatgattgtttctatctcttgtgaatccacttttcagagtttcgtaaaattatcaatgtttgtcatctacatgagttctctgatgcataatgagctgtgacttccaacaaaaggctttcccacattcagtgcacttacaaggcttctctcctgtatgtgttctctgatgtgcactgagaattgatttttgagagaaggttttcccacattcattgcacccatagggtttctctcctgaatgagttctttgatgtacaatgagttgagaattcctaatgaaggcttttccacactcactgcattcatatggtttctctcttgtgtgcattctctggtgtacaagaaggcgtaatttcccactgaaggatttctcacattgactgcatttataagggttgacccctgcatgagttcgctcatgtacaatgagtagtgatttccaaatgaaggctttcccacattcattacattcatatggtttttcacctgaatgagttctcatgtgtataattaggtatgacttgctgctaaaagctttcccacattcactgcacccataaggcttttcccctgcatgagttcgctgatgtgaaatgagctggtctttcctattaaaggctttcccacattcactgcattcatagggattttctcctgtgtgaattctctgatgcacaatgagttgtgaattgaaactaaaggatttcccgcattccctgcactcatgtggtttctctcctgtatgagttctcatatgtataataaggtatgacttgctcctgaaggctttcccacactcactgcatccatatggttttactcctgtgtgacttctctgatgtacaatgagctgggacttcaaactaaaggtttttgcacattgactgcatccatagggttttactccagtgtgcactcctttatgtacaatgagctgtgatttgaacgtaaaggcttttccacattcattacaactatagggtttctctcctgtatgagttctctgatgtacaatcaggtttgactttgtattaaaggctttctgacactcactacattcaaatggtttctcccctgtatgagttctctggtgtataataagctgtgactttaaaccaaaagcctttccacagtcggtgcattcataaggcttctctcctgcatgagttctctggtgtgaaataagctggtatttccgactgaaggctttcccacattcatggcattcataggggttctctcctgtatgaatcctctgatgtataatgagctgtgatttaaaactgaaggctttcccacaattgttgcattcatggagtttttctcctgtatgagtccttgtatgtataataaggtatgacttgctcctgaaggctttgccacattcattgcatacataaggtttcattcctgtgtgacttctctgatgtacaatgagctgtgatttcaaactgaatcctttaccacactgaatacacccatagggctttactcctgtgtgaatcccctgatgtacaatgagctgtgacttgaatgtaaaggcttttccacaatcactacaaacataaggtttctcccctgtatgggttctctgatgtaccataaggtttgactttgtattaaaggctttctgacattcattgcattcatatggtttctctcctgtatgaattctttcatgtataatgagctgtgattttaaaccaaaagctttcccacattcattacacacatatggtttctgtcctgaatgagttttctggtgtgaaacaagctggtctttcctactgaagactttcccacattcacagcactcatagggattctcacctgtgtgaattctctgatgtataacaagctgtgaatggaaactgaatgttttcctgcattcactgcattcatgtagtttctctcctgtatgaattctctgatgtacaatgaggtatgatttactactgaagtctttcccacattcattacaaccatagggtttctcttcggcatgagtttgctgatgcactagaaggtatgacttgctgctgaaggctttctcacaacagctgcatccaaagggtttttcgcccatatacatttgttggcacataagttgcgatttcttattgacggtttttccagattcaatactttcacagtattttattccaataacagtttgctcatgtttagaatggaagaatgattttccatgtacctgaaacccattaggattatttctagcataatcactagtgaaatctatatatttcaaactctttccatgcgtgccacatttatgaggtttttgtcttgaaagatactttgtactaagaagacatagttttccaaatgtagtgcattcaaagctttttgccgtacttcccagcttgtctttattttcctgatgccaatccataagatcatcaattttccagactgtgtccaggacttggtgatttttggctgctcttgggaaataaacagccactctaggactttctctattctgcgactcttctgcttctgcctgggtgttccagggagaggttgcagaccaggagtcccttggcccaagatggattcctgaccttggagctttctgatcctatcccatgaactgtttcgttcttggagaggtgggacccaaatagaagctgtccggaccctggtggccatccctacggtcagttttgtgtgcctcgctggaagtgacaggacgcgagggatgctccggctcctccaaaccctgaaggggcagcagaatagagtccagggtactgcctccacctccagatctgcagccagaagggttcgcaaccactccagactcggctggcccgttgaccacgacgggcgatgaacgctatctgaggaacaaggatctcgccatcggcgcggaacaatggcggccgctacgtat

SEQ ID NO: 18790 - RNA, 12583 nt, Homo sapiens
  source 1..12583: mol_type = other RNA
tgatatgtttgatattgggttgtctttttgttgttgggttgtaagagttctttatatgttctggatactagacccttatcaggtatattattttacagtgtcttttctcctatattcaccttttttttttttgagacggagtctcgctctgtcgcccaggctggagtgcagtggtgagatctgggctcactggttccaggttcacgccattctccttcctcagcctcccaagtagctgggactacaggcttccactaccagcctggctaattttttgtatttttttgtagagacagggtttcaccacattagccaggatggtttcgatctcctgacctcgtgatccacctgcctcagcctcccaaagtgctaggattacaggcgtgagccaccacacccggccttttttttttttttgagatggaattttgctttcttgctctgtcacctgggctggagtgcagtagcatgatctcggctcactgcaacctccacctcacagcttcaagcgatcctcctgcctcagcttcctgagttgctgggattacaggcacatgccaccacacccggcttttttttttctctttttttttatttttagtagagacgtggtttcaccaagttaaccaggctggtctcgcactcctgacctcaagtgatcctcccaccttggcctcccaaagtgctggaattacaggcgtgagccaccacacccagctccttttcactttcttgatagtgtccactgatgccgaaagttttcaattttggtgaagtccaatttacctattttttcttttgtttcccatgcttctggtgtcatatccaataaatcattgccaaatccagtgccaagaagtacatgaaaagattttcaacatcactagccattaggtaaaggaaaatcaaaaccacaatgagataccatttcatacatgttagagtggctattataaaaaatatggaggccaagtgcagtggttcaagcctgtaatcccagcactttgggaggccaaggtaagtggatcacttgaggacaggagtttgagactagcctggcctggccaacatggtgaaaccctgtctctactaaaaatacaaaaaatagccatacatggtggcacatgcctgtaatcccagctactcaggaggccgaggaaggagaatcacttaaacctaggaggcggaggttgcagtgagctgaaatggtgccactgcactccagcctgggtgacagagtgaaactccatttcaaaaaaaccaaaaaactatttgggtgtagtggcacctgtagttccagctacccaggaggctgaggtggaaggatcccttgagcccaggaggttggggctgcagtgagttatgatcatgcctatgaaatgagagagaaacaaactaattaatattggcaagtatgtggagaaattggaagccttgtgcactgctggtggaatgtaaaatgatagttgcacaataatggaaataatgtacttcatgccactgaagtgtacacttaaaaatagttaaaatggtaaatgttcttattatatatatgtgtatatatatgtgtatatgtgtatatatatgtgtatatatgtgtgtatgtgtgtgtgtatatatacatatatatatatatatatatatatatatatatatatatatatatatatatataaaatcacacatgaaagtctcccttggaactgatcctgaaataatttcatgtgtgatgaaagaacaccctgctctcctggagtgataagtggcctttttgttcatgctggcattatacatcccaggctcttccacacacacccagcataatttcaccaagcagagggagtacactctccaaaggcccatttgtgcctgtttctatcattatatcctcctatttaactcactccctgccctctacaaaccgtcatcaatcacagatatgtttgctacccctgtagtttctgcttttccataacatcatagaaataggatcatacagccttttcacactggtctctttcacttagcaatatgcctatcagattcatccatgtcctgcatggcctcagagcttgctcttgctgaacaggactccattgcatggatgtaccccagcctagttagtcattcacctattgaaggttatcctgattccttaaagtatttgtctgttatgaaaagagctgctgtacgtgagtacatgctgggttttgtttagatcaaactcctatgttttcaaagcagttatctaaatacctaggagtgtgattgttggctcatattgtgaagctttgtttagctttggggaaaagtcaaactatcttccaaagtggctatactattatgcattgcaccagcaatgaatgagagttcctgttgcaattgcaaatttacttatttttagattatagtcactttaatagatgtgcggtgctatctcgttgttttaatttgcttttccctcatgacaagtgtcactgagcattatttggtatgcttatttgccatctgtatatcttcttttttttttttttgagacggagtttcactcttgttgcccaggctggagtgcaatggcgcgatctcggctcacagcaacctccgcctcccgggttcaagccattctcctgcctccgcctccggagtagctaccacttggtggcagagtagcgccaccacgcctggctaattttgtatttttagtagagacagggtttctccatgttggtcaggctggtctcgaactccggacctcaggtgatctgcccgcctcggcctcccaaagtgctgggattacaggcgtgagccaccgtgcctggccaccatctgtatatctttggaaagtatgtatttggatctgtccccatttttaattgggttgtcttcttgttcaattttagggttttttttttatattttgcatacaaacactttttcagatttttttgaatgattttattcattacaaattccaattattgctatacattatttcaaatatataggaaatcacttgacttttgtctatggccatctactttgccttttattatctctatccattccaattaaggcatggaatgatggactctatttcagtttcgttttccaaaattatggcatggaaaatcgtaagattgaatttcaggggttcactgggactgcaagagggggcacatggccatcacaaaacaggaagcactgaccatccaacactgtgcctaggtagtaaggaaggggtgcaagcacacaccttgtctagcctgcttgcagtacctgcattctgctcacagacctctgggttgaatccacagaggaccaggccttccttctactcaggacctggggatcactagaggctgcatcacagtaaagactgagctgccttctcctcaggactgacctggggacccttggcaggggggaatccacagtgacaaacagaccttgcttctactcaggacccggagacccccgagggcacttcacagtgatgaccagaatttacctcatctcaggaccaacctgggggatgcatcacactgagaaccagagcttccttctccactggccaacctgaggaccactgtggggcacaaccacagtgaagactggagcttgtttctcttcaggactgacctagggaccctagtggggcaaatccacagtgaggttctgagcttccttctcctcaggaccaacctggggacccctgggaggtagatcacagtgatgaccagagtatcctcctcaggactgacccgtggtgggggatgcaaccacagtgaggactaaagcttccttttcctcacaacctggggaccccctagggggatacatcacagtgagatccagagcttccatatctgaagactcctgtagggtacacccacagtgacgaccagtgcactttccggaccaatctggggcgatgtcatctcacctttgggatacatggaggccacaggaggaaaagatgaggaaaagtgaggcctgcaccctgagtgctgaggagggagctttgctgtttcactttgccctgtaatatctgaacaagatttattttaggaaatcgtacctctattgaggtttccactagtcatctttatagcaagcccaactactttttatacatatgggtttgtttctggggagaaatcccagtacaaaaaaagggagaaacactgcgacaaaacactgcaacagtccaggtcaaagttggggatgaacagcacctgtgggatcaccctggatcccaagagggaagggcaaatgtgcaccctatgtgcttgcttttattaattttttttgaaggagtctcactctgctgcccgggctggagtgcaatggcacaatctcagctcactgcaacctccgcctctccagttcaagcaattctcctgagtagcttggattatagatgcatgccaccacagctggccaatttttgtatttttagtagagacggggtttcaccaggctggtctcgaactcctgacctcaagtcatccacctgcctcagcctcacaaaatgctgagattacaggcatgagccaccatgcccagcctttttattaatgttttaatggcctgtgtttctaacaagtagttgaaacaatgttgaaaattaaagagtagacatgttaaaacttgcaacttcatttaaatttaaatatatcatttataccaaaatcagaatttatttaagatttatggctgggtgcttggctcacacctgtaatcctagcactttgggaggccaaggcaggtggactgcttgagcccaggagtttgaaaccagactggaaaacatggtaaaaccccatctctacaagaaataaataactctacctggccctttagcaaagaattaagaaaaatcaatacagaccagtggctcacacctgtaatcccagcactttgggaggctgagggtggatcacgaggtcaggagttcaagaccagcctggccaacatggtgaaaccccatctctactaaaaacacaaaaattagctgggcgtggtggcgtgtgcctgtaattccagctactagggaggctgaggcaggagaattgcttgaacccaggaggcagaggttgcagtgagccaagaacacaccactgcactccagcctggcaatacagcgagactccatctcaaaaaaaaaaaaaaaaatgcaaatactatgccatataaggagcttgagcatccacagggagtatctgtggttgcgggggggtcctccatgaatactgacaactgcatacttgctactctactggcagttccaaacatttgtttgtggtttattttgggtttcctaattacacgatcacatctccaattcatggcagttgtttctgcacccatccctaattcctcacattccttgttttcacaccttggctagatgttactcatttcataaaagtgatgcgcattcttgtaattttgctttgttttttacagacagggtctcactttgttgcccaggatggagtgcaggggcatgatcatagctcactgtagccttgaactactggactcaagctaacctcctgcctcagcctcctcagtaggtgggactaccggcacttgccactacacctggctgatcttttttttgagatggaggcttgttctgtcgcccagcctggagtgcagtggtgcaatcttggctcactgcaactgccacctcctaggttcaagcaattcttctgcctcagcctcccgagtagatgggattacaggcacgtgccaccacacctggctgacttttgtatttttagtagagacggggtttcaccatgttagccacactggtcttgaaatcctgacctcaagtgatctgcccacctcggcctcccaaagtgctgggattacaggcatgagccacggcgcctgaccacacctggctaatctttttaaaaagtttttgtacagacagggtctccctatattggtcaggcttgtctcgaactcctgggttccagcaatcctccagcctcagccttcccaagtgctggtattacatggatgagccactgcacctggctaattttactttaaaggaatctttctactattttatcattaagtatgacatttgtgttttcagaacatatattccctaccaagttacaggagttaattttaattcccaacttaatagtattttagtgtcatctatgggtgttaaattccatcaagtgatttatcagcatatactgagataatccttatgagttttatctggtagttaattaaaatattttctaatattaaatcttccaaacatactcttctgttttttgagacagggtctagttctgtcacccagggtggagtacagtggtacgatctcagctcactgcaacttccgcctcctagattcaagtgattctcccgtcccagcctcccaagtagctgggattataggtgtcagttaccatgccctgctatttttttgtatttttagtagagaggggtttcaccatgttggccaggctggtctcaaactcctgacctcaggtgatccaccatctcagcctcctgaagtgctgggattataggtgtgagccaccgtgcctggccccatatatctctttttaagtgggcatactgccattataaataatagtgattctgctggtaatgaacaaaggatgctggatccactaatagtctgttaaacctaatatcatgactttcttgttagctatacattggtttgctataattccatttagaatttttaaacctatgttcacaaatatggatttttaaacctatgttcacaaatatggatttttaaacctatgttcacaaatatggtttgcaagtcattttttctcctaaatttctatttgatggggaagttgtaaaatattggggttatttttccttggattttccttataataactattcctgaaaagtctctggaatgtctttcttttctggggctggggtagaaggactagatagatttacaaaccagtaactcaatttctgttttgtaaaattttcatttcattaaataataagtcctaatcaagtattattctttcccacagtatgtgagtgctgtcctcaatactgtcaacacttctggcttctaccaggcaaggctgcatgtagatttgcatctgaaaaaacaacaaactaaaatctaaccctaggtagtagtaaactgaatataaactttctcttatgaatttattctgtcttctttggtacatcaataataatatacacctttacagtatttcccagattgggggatacactttagcaagtatctgcgattatttgtttatgtaagatgtcccttcccttctgtgaatcatcattcttcaccccaagtatcttgagattggattctgtataagcagaatacaacagttaggcattcaggtatcattaaattcctccgcttcaaggatgaaaatttctttgggtatctaatagagtacaaagcagaaggtgtttcagaaatatttgcagtattgaatccgcatattcctccaagatagccctaatctaactggcagggtcccactcttcccagattaatgcccactcacataacaaacctgatgaggtagtgaagaaaactaactttgtgagtaagcaactggcagagtttttcaccactgtgactctatagctacatgtaactaagtagtatcactgacacataatcttaaattgaagttttaagatcattattctccatgttatacatgggtatcaaaagcattcccctcttgaccactccagaattctgtttaaaatttttcaatgacaacttatccatttccccaaagcctcagtgagcacatgatgccaacaattcatttcatgacttcatagcatgggccaagtttcttgcttaaaagacttccatcctgtcttgggaaacaaccatttccaaatatccacatatccttgcaagtttctgcctactcctctaccacccatttctgaagccatctgatttagtaagctgtatgcaaaagatacacaatggctaatgcaatcaaacaaggaatgtattaaaagcacacccaatagctcaaaataaaagacaagtgaacaaagttaagaaaatgacagtaacaaaagctgttctgggaacctctattgaaatagctacttattacatcaacatgctaccacagaacaaaagctcatgttgcttttctgaacttgaaaaacccattaacaatgtacagttctgagcctcagctgaccatagtgctcatgccaagtcctgagcagggcatcttgaatggtggttccctcatgactacatacaccgttagggaatgtttcgttaagaggaaatcaagatgttctaacctgtgaaggtagaatagattccaggctacacaaacacatgaagtgtgccttatattgattactaaagaggttgctgccaagactgcttccaaagggcagaagatagccctaaaaaatgtttgcagtgtggaaatgcatttttagtaagtcatattctagtaacaagttgcatttggtaagacacaaagaaacaatgttggtatgcagagtagaaatctctggaagatgatattgtcatatcagagatattgtcagtatcagagatactgaaatctctggaagatgatttttgtctcacatatggcattcgcaagtaaaatgccaaactgcaaaattcatattatgtagtacacataggaagatatctaaatatccctgtaggctctgggatgttatttcttattcttaacctccttactagattcacttgtacaatgaaataatctgtatcttattatttataattgagaattttctcaaaccttttcctgaaattttggaacacctggaataaaatttcttaaaatgattcctaaaagaaataattcttcaaaattaatattaagatataataacaggttggtttttttttttttttttttttttttttttagaatgaagcttctaaggtgaggttaacagtccagctgtggtttatttggtacattcataagatgttcactcctatatatattttttccctaggggtttctcatttctagatttacactttcccttatagcatggtccctccaaggtatatgcttccgatacataaaatgtttgtaattttgttaattctgccattcattagctcaataatttctctcattaaaattctgtaaactatgaatttcaaagaagtctattctatattcatctggttcatgaagtttcctctttgtgaatcttattttagtaaaatgactttacaacgtttaacatggttcctcacctgtatgaactttttaaaaaaaggtatgacttgctgctaaaaattttcagagtggttactaaattcagttttcctgtgtattgtctactatctttttgcatgtaaagaacagctttctgtggatgcctttccatatgctgtgcattcataaagtttctattcagtatgagttttctggaagatgacaagatgattccacttacagagtttctctttatatatgattgtttctatctcttgtgaatccacttttcagagtttcgtaaaattatcaatgtttgtcatctacatgagttctctgatgcataatgagctgtgacttccaacaaaaggctttcccacattcagtgcacttacaaggcttctctcctgtatgtgttctctgatgtgcactgagaattgatttttgagagaaggttttcccacattcattgcacccatagggtttctctcctgaatgagttctttgatgtacaatgagttgagaattcctaatgaaggcttttccacactcactgcattcatatggtttctctcttgtgtgcattctctggtgtacaagaaggcgtaatttcccactgaaggatttctcacattgactgcatttataagggttgacccctgcatgagttcgctcatgtacaatgagtagtgatttccaaatgaaggctttcccacattcattacattcatatggtttttcacctgaatgagttctcatgtgtataattaggtatgacttgctgctaaaagctttcccacattcactgcacccataaggcttttcccctgcatgagttcgctgatgtgaaatgagctggtctttcctattaaaggctttcccacattcactgcattcatagggattttctcctgtgtgaattctctgatgcacaatgagttgtgaattgaaactaaaggatttcccgcattccctgcactcatgtggtttctctcctgtatgagttctcatatgtataataaggtatgacttgctcctgaaggctttcccacactcactgcatccatatggttttactcctgtgtgacttctctgatgtacaatgagctgggacttcaaactaaaggtttttgcacattgactgcatccatagggttttactccagtgtgcactcctttatgtacaatgagctgtgatttgaacgtaaaggcttttccacattcattacaactatagggtttctctcctgtatgagttctctgatgtacaatcaggtttgactttgtattaaaggctttctgacactcactacattcaaatggtttctcccctgtatgagttctctggtgtataataagctgtgactttaaaccaaaagcctttccacagtcggtgcattcataaggcttctctcctgcatgagttctctggtgtgaaataagctggtatttccgactgaaggctttcccacattcatggcattcataggggttctctcctgtatgaatcctctgatgtataatgagctgtgatttaaaactgaaggctttcccacaattgttgcattcatggagtttttctcctgtatgagtccttgtatgtataataaggtatgacttgctcctgaaggctttgccacattcattgcatacataaggtttcattcctgtgtgacttctctgatgtacaatgagctgtgatttcaaactgaatcctttaccacactgaatacacccatagggctttactcctgtgtgaatcccctgatgtacaatgagctgtgacttgaatgtaaaggcttttccacaatcactacaaacataaggtttctcccctgtatgggttctctgatgtaccataaggtttgactttgtattaaaggctttctgacattcattgcattcatatggtttctctcctgtatgaattctttcatgtataatgagctgtgattttaaaccaaaagctttcccacattcattacacacatatggtttctgtcctgaatgagttttctggtgtgaaacaagctggtctttcctactgaagactttcccacattcacagcactcatagggattctcacctgtgtgaattctctgatgtataacaagctgtgaatggaaactgaatgttttcctgcattcactgcattcatgtagtttctctcctgtatgaattctctgatgtacaatgaggtatgatttactactgaagtctttcccacattcattacaaccatagggtttctcttcggcatgagtttgctgatgcactagaaggtatgacttgctgctgaaggctttctcacaacagctgcatccaaagggtttttcgcccatatacatttgttggcacataagttgcgatttcttattgacggtttttccagattcaatactttcacagtattttattccaataacagtttgctcatgtttagaatggaagaatgattttccatgtacctgaaacccattaggattatttctagcataatcactagtgaaatctatatatttcaaactctttccatgcgtgccacatttatgaggtttttgtcttgaaagatactttgtactaagaagacatagttttccaaatgtagtgcattcaaagctttttgccgtacttcccagcttgtctttattttcctgatgccaatccataagatcatcaattttccagactgtgtctccagaggatgcagcaacaaggcgtcatcttggaagcacagagcaggccctcaccagacaccaaacctgccagcaccttggctttggactttccagccttcaaaattggacaggtctgatttggaacttgggcctgcaccatacacagctcttctccttgttccaacttgaagatgatatcaggtttggtgtgttggtaccctagggacaccaggttgctatagttctccaacatcacactcctgtacaggcacttctgtgctgggtctagcagctgccactcctcccaggtaaaatccacaaacacatccatgaatgacaaaggtccccaaatagaagctgtccggaccctggtggccatccctacggtcagttttgtgtgcctcgctggaagtgacaggacgcgagggatgctccggctcctccaaaccctgaaggggcagcagaatagagtccagggtactgcctccacctccagatctgcagccagaagggttcgcaaccactccagactcggctggcccgttgaccacgacgggcgatgaacgctatctgaggaacaaggatctcgccatcggcgcggaacaatggcggccgctacgtat

SEQ ID NO: 18791 - RNA, 12784 nt, Homo sapiens
  source 1..12784: mol_type = other RNA
tgatatgtttgatattgggttgtctttttgttgttgggttgtaagagttctttatatgttctggatactagacccttatcaggtatattattttacagtgtcttttctcctatattcaccttttttttttttgagacggagtctcgctctgtcgcccaggctggagtgcagtggtgagatctgggctcactggttccaggttcacgccattctccttcctcagcctcccaagtagctgggactacaggcttccactaccagcctggctaattttttgtatttttttgtagagacagggtttcaccacattagccaggatggtttcgatctcctgacctcgtgatccacctgcctcagcctcccaaagtgctaggattacaggcgtgagccaccacacccggccttttttttttttttgagatggaattttgctttcttgctctgtcacctgggctggagtgcagtagcatgatctcggctcactgcaacctccacctcacagcttcaagcgatcctcctgcctcagcttcctgagttgctgggattacaggcacatgccaccacacccggcttttttttttctctttttttttatttttagtagagacgtggtttcaccaagttaaccaggctggtctcgcactcctgacctcaagtgatcctcccaccttggcctcccaaagtgctggaattacaggcgtgagccaccacacccagctccttttcactttcttgatagtgtccactgatgccgaaagttttcaattttggtgaagtccaatttacctattttttcttttgtttcccatgcttctggtgtcatatccaataaatcattgccaaatccagtgccaagaagtacatgaaaagattttcaacatcactagccattaggtaaaggaaaatcaaaaccacaatgagataccatttcatacatgttagagtggctattataaaaaatatggaggccaagtgcagtggttcaagcctgtaatcccagcactttgggaggccaaggtaagtggatcacttgaggacaggagtttgagactagcctggcctggccaacatggtgaaaccctgtctctactaaaaatacaaaaaatagccatacatggtggcacatgcctgtaatcccagctactcaggaggccgaggaaggagaatcacttaaacctaggaggcggaggttgcagtgagctgaaatggtgccactgcactccagcctgggtgacagagtgaaactccatttcaaaaaaaccaaaaaactatttgggtgtagtggcacctgtagttccagctacccaggaggctgaggtggaaggatcccttgagcccaggaggttggggctgcagtgagttatgatcatgcctatgaaatgagagagaaacaaactaattaatattggcaagtatgtggagaaattggaagccttgtgcactgctggtggaatgtaaaatgatagttgcacaataatggaaataatgtacttcatgccactgaagtgtacacttaaaaatagttaaaatggtaaatgttcttattatatatatgtgtatatatatgtgtatatgtgtatatatatgtgtatatatgtgtgtatgtgtgtgtgtatatatacatatatatatatatatatatatatatatatatatatatatatatatatatataaaatcacacatgaaagtctcccttggaactgatcctgaaataatttcatgtgtgatgaaagaacaccctgctctcctggagtgataagtggcctttttgttcatgctggcattatacatcccaggctcttccacacacacccagcataatttcaccaagcagagggagtacactctccaaaggcccatttgtgcctgtttctatcattatatcctcctatttaactcactccctgccctctacaaaccgtcatcaatcacagatatgtttgctacccctgtagtttctgcttttccataacatcatagaaataggatcatacagccttttcacactggtctctttcacttagcaatatgcctatcagattcatccatgtcctgcatggcctcagagcttgctcttgctgaacaggactccattgcatggatgtaccccagcctagttagtcattcacctattgaaggttatcctgattccttaaagtatttgtctgttatgaaaagagctgctgtacgtgagtacatgctgggttttgtttagatcaaactcctatgttttcaaagcagttatctaaatacctaggagtgtgattgttggctcatattgtgaagctttgtttagctttggggaaaagtcaaactatcttccaaagtggctatactattatgcattgcaccagcaatgaatgagagttcctgttgcaattgcaaatttacttatttttagattatagtcactttaatagatgtgcggtgctatctcgttgttttaatttgcttttccctcatgacaagtgtcactgagcattatttggtatgcttatttgccatctgtatatcttcttttttttttttttgagacggagtttcactcttgttgcccaggctggagtgcaatggcgcgatctcggctcacagcaacctccgcctcccgggttcaagccattctcctgcctccgcctccggagtagctaccacttggtggcagagtagcgccaccacgcctggctaattttgtatttttagtagagacagggtttctccatgttggtcaggctggtctcgaactccggacctcaggtgatctgcccgcctcggcctcccaaagtgctgggattacaggcgtgagccaccgtgcctggccaccatctgtatatctttggaaagtatgtatttggatctgtccccatttttaattgggttgtcttcttgttcaattttagggttttttttttatattttgcatacaaacactttttcagatttttttgaatgattttattcattacaaattccaattattgctatacattatttcaaatatataggaaatcacttgacttttgtctatggccatctactttgccttttattatctctatccattccaattaaggcatggaatgatggactctatttcagtttcgttttccaaaattatggcatggaaaatcgtaagattgaatttcaggggttcactgggactgcaagagggggcacatggccatcacaaaacaggaagcactgaccatccaacactgtgcctaggtagtaaggaaggggtgcaagcacacaccttgtctagcctgcttgcagtacctgcattctgctcacagacctctgggttgaatccacagaggaccaggccttccttctactcaggacctggggatcactagaggctgcatcacagtaaagactgagctgccttctcctcaggactgacctggggacccttggcaggggggaatccacagtgacaaacagaccttgcttctactcaggacccggagacccccgagggcacttcacagtgatgaccagaatttacctcatctcaggaccaacctgggggatgcatcacactgagaaccagagcttccttctccactggccaacctgaggaccactgtggggcacaaccacagtgaagactggagcttgtttctcttcaggactgacctagggaccctagtggggcaaatccacagtgaggttctgagcttccttctcctcaggaccaacctggggacccctgggaggtagatcacagtgatgaccagagtatcctcctcaggactgacccgtggtgggggatgcaaccacagtgaggactaaagcttccttttcctcacaacctggggaccccctagggggatacatcacagtgagatccagagcttccatatctgaagactcctgtagggtacacccacagtgacgaccagtgcactttccggaccaatctggggcgatgtcatctcacctttgggatacatggaggccacaggaggaaaagatgaggaaaagtgaggcctgcaccctgagtgctgaggagggagctttgctgtttcactttgccctgtaatatctgaacaagatttattttaggaaatcgtacctctattgaggtttccactagtcatctttatagcaagcccaactactttttatacatatgggtttgtttctggggagaaatcccagtacaaaaaaagggagaaacactgcgacaaaacactgcaacagtccaggtcaaagttggggatgaacagcacctgtgggatcaccctggatcccaagagggaagggcaaatgtgcaccctatgtgcttgcttttattaattttttttgaaggagtctcactctgctgcccgggctggagtgcaatggcacaatctcagctcactgcaacctccgcctctccagttcaagcaattctcctgagtagcttggattatagatgcatgccaccacagctggccaatttttgtatttttagtagagacggggtttcaccaggctggtctcgaactcctgacctcaagtcatccacctgcctcagcctcacaaaatgctgagattacaggcatgagccaccatgcccagcctttttattaatgttttaatggcctgtgtttctaacaagtagttgaaacaatgttgaaaattaaagagtagacatgttaaaacttgcaacttcatttaaatttaaatatatcatttataccaaaatcagaatttatttaagatttatggctgggtgcttggctcacacctgtaatcctagcactttgggaggccaaggcaggtggactgcttgagcccaggagtttgaaaccagactggaaaacatggtaaaaccccatctctacaagaaataaataactctacctggccctttagcaaagaattaagaaaaatcaatacagaccagtggctcacacctgtaatcccagcactttgggaggctgagggtggatcacgaggtcaggagttcaagaccagcctggccaacatggtgaaaccccatctctactaaaaacacaaaaattagctgggcgtggtggcgtgtgcctgtaattccagctactagggaggctgaggcaggagaattgcttgaacccaggaggcagaggttgcagtgagccaagaacacaccactgcactccagcctggcaatacagcgagactccatctcaaaaaaaaaaaaaaaaatgcaaatactatgccatataaggagcttgagcatccacagggagtatctgtggttgcgggggggtcctccatgaatactgacaactgcatacttgctactctactggcagttccaaacatttgtttgtggtttattttgggtttcctaattacacgatcacatctccaattcatggcagttgtttctgcacccatccctaattcctcacattccttgttttcacaccttggctagatgttactcatttcataaaagtgatgcgcattcttgtaattttgctttgttttttacagacagggtctcactttgttgcccaggatggagtgcaggggcatgatcatagctcactgtagccttgaactactggactcaagctaacctcctgcctcagcctcctcagtaggtgggactaccggcacttgccactacacctggctgatcttttttttgagatggaggcttgttctgtcgcccagcctggagtgcagtggtgcaatcttggctcactgcaactgccacctcctaggttcaagcaattcttctgcctcagcctcccgagtagatgggattacaggcacgtgccaccacacctggctgacttttgtatttttagtagagacggggtttcaccatgttagccacactggtcttgaaatcctgacctcaagtgatctgcccacctcggcctcccaaagtgctgggattacaggcatgagccacggcgcctgaccacacctggctaatctttttaaaaagtttttgtacagacagggtctccctatattggtcaggcttgtctcgaactcctgggttccagcaatcctccagcctcagccttcccaagtgctggtattacatggatgagccactgcacctggctaattttactttaaaggaatctttctactattttatcattaagtatgacatttgtgttttcagaacatatattccctaccaagttacaggagttaattttaattcccaacttaatagtattttagtgtcatctatgggtgttaaattccatcaagtgatttatcagcatatactgagataatccttatgagttttatctggtagttaattaaaatattttctaatattaaatcttccaaacatactcttctgttttttgagacagggtctagttctgtcacccagggtggagtacagtggtacgatctcagctcactgcaacttccgcctcctagattcaagtgattctcccgtcccagcctcccaagtagctgggattataggtgtcagttaccatgccctgctatttttttgtatttttagtagagaggggtttcaccatgttggccaggctggtctcaaactcctgacctcaggtgatccaccatctcagcctcctgaagtgctgggattataggtgtgagccaccgtgcctggccccatatatctctttttaagtgggcatactgccattataaataatagtgattctgctggtaatgaacaaaggatgctggatccactaatagtctgttaaacctaatatcatgactttcttgttagctatacattggtttgctataattccatttagaatttttaaacctatgttcacaaatatggatttttaaacctatgttcacaaatatggatttttaaacctatgttcacaaatatggtttgcaagtcattttttctcctaaatttctatttgatggggaagttgtaaaatattggggttatttttccttggattttccttataataactattcctgaaaagtctctggaatgtctttcttttctggggctggggtagaaggactagatagatttacaaaccagtaactcaatttctgttttgtaaaattttcatttcattaaataataagtcctaatcaagtattattctttcccacagtatgtgagtgctgtcctcaatactgtcaacacttctggcttctaccaggcaaggctgcatgtagatttgcatctgaaaaaacaacaaactaaaatctaaccctaggtagtagtaaactgaatataaactttctcttatgaatttattctgtcttctttggtacatcaataataatatacacctttacagtatttcccagattgggggatacactttagcaagtatctgcgattatttgtttatgtaagatgtcccttcccttctgtgaatcatcattcttcaccccaagtatcttgagattggattctgtataagcagaatacaacagttaggcattcaggtatcattaaattcctccgcttcaaggatgaaaatttctttgggtatctaatagagtacaaagcagaaggtgtttcagaaatatttgcagtattgaatccgcatattcctccaagatagccctaatctaactggcagggtcccactcttcccagattaatgcccactcacataacaaacctgatgaggtagtgaagaaaactaactttgtgagtaagcaactggcagagtttttcaccactgtgactctatagctacatgtaactaagtagtatcactgacacataatcttaaattgaagttttaagatcattattctccatgttatacatgggtatcaaaagcattcccctcttgaccactccagaattctgtttaaaatttttcaatgacaacttatccatttccccaaagcctcagtgagcacatgatgccaacaattcatttcatgacttcatagcatgggccaagtttcttgcttaaaagacttccatcctgtcttgggaaacaaccatttccaaatatccacatatccttgcaagtttctgcctactcctctaccacccatttctgaagccatctgatttagtaagctgtatgcaaaagatacacaatggctaatgcaatcaaacaaggaatgtattaaaagcacacccaatagctcaaaataaaagacaagtgaacaaagttaagaaaatgacagtaacaaaagctgttctgggaacctctattgaaatagctacttattacatcaacatgctaccacagaacaaaagctcatgttgcttttctgaacttgaaaaacccattaacaatgtacagttctgagcctcagctgaccatagtgctcatgccaagtcctgagcagggcatcttgaatggtggttccctcatgactacatacaccgttagggaatgtttcgttaagaggaaatcaagatgttctaacctgtgaaggtagaatagattccaggctacacaaacacatgaagtgtgccttatattgattactaaagaggttgctgccaagactgcttccaaagggcagaagatagccctaaaaaatgtttgcagtgtggaaatgcatttttagtaagtcatattctagtaacaagttgcatttggtaagacacaaagaaacaatgttggtatgcagagtagaaatctctggaagatgatattgtcatatcagagatattgtcagtatcagagatactgaaatctctggaagatgatttttgtctcacatatggcattcgcaagtaaaatgccaaactgcaaaattcatattatgtagtacacataggaagatatctaaatatccctgtaggctctgggatgttatttcttattcttaacctccttactagattcacttgtacaatgaaataatctgtatcttattatttataattgagaattttctcaaaccttttcctgaaattttggaacacctggaataaaatttcttaaaatgattcctaaaagaaataattcttcaaaattaatattaagatataataacaggttggtttttttttttttttttttttttttttttagaatgaagcttctaaggtgaggttaacagtccagctgtggtttatttggtacattcataagatgttcactcctatatatattttttccctaggggtttctcatttctagatttacactttcccttatagcatggtccctccaaggtatatgcttccgatacataaaatgtttgtaattttgttaattctgccattcattagctcaataatttctctcattaaaattctgtaaactatgaatttcaaagaagtctattctatattcatctggttcatgaagtttcctctttgtgaatcttattttagtaaaatgactttacaacgtttaacatggttcctcacctgtatgaactttttaaaaaaaggtatgacttgctgctaaaaattttcagagtggttactaaattcagttttcctgtgtattgtctactatctttttgcatgtaaagaacagctttctgtggatgcctttccatatgctgtgcattcataaagtttctattcagtatgagttttctggaagatgacaagatgattccacttacagagtttctctttatatatgattgtttctatctcttgtgaatccacttttcagagtttcgtaaaattatcaatgtttgtcatctacatgagttctctgatgcataatgagctgtgacttccaacaaaaggctttcccacattcagtgcacttacaaggcttctctcctgtatgtgttctctgatgtgcactgagaattgatttttgagagaaggttttcccacattcattgcacccatagggtttctctcctgaatgagttctttgatgtacaatgagttgagaattcctaatgaaggcttttccacactcactgcattcatatggtttctctcttgtgtgcattctctggtgtacaagaaggcgtaatttcccactgaaggatttctcacattgactgcatttataagggttgacccctgcatgagttcgctcatgtacaatgagtagtgatttccaaatgaaggctttcccacattcattacattcatatggtttttcacctgaatgagttctcatgtgtataattaggtatgacttgctgctaaaagctttcccacattcactgcacccataaggcttttcccctgcatgagttcgctgatgtgaaatgagctggtctttcctattaaaggctttcccacattcactgcattcatagggattttctcctgtgtgaattctctgatgcacaatgagttgtgaattgaaactaaaggatttcccgcattccctgcactcatgtggtttctctcctgtatgagttctcatatgtataataaggtatgacttgctcctgaaggctttcccacactcactgcatccatatggttttactcctgtgtgacttctctgatgtacaatgagctgggacttcaaactaaaggtttttgcacattgactgcatccatagggttttactccagtgtgcactcctttatgtacaatgagctgtgatttgaacgtaaaggcttttccacattcattacaactatagggtttctctcctgtatgagttctctgatgtacaatcaggtttgactttgtattaaaggctttctgacactcactacattcaaatggtttctcccctgtatgagttctctggtgtataataagctgtgactttaaaccaaaagcctttccacagtcggtgcattcataaggcttctctcctgcatgagttctctggtgtgaaataagctggtatttccgactgaaggctttcccacattcatggcattcataggggttctctcctgtatgaatcctctgatgtataatgagctgtgatttaaaactgaaggctttcccacaattgttgcattcatggagtttttctcctgtatgagtccttgtatgtataataaggtatgacttgctcctgaaggctttgccacattcattgcatacataaggtttcattcctgtgtgacttctctgatgtacaatgagctgtgatttcaaactgaatcctttaccacactgaatacacccatagggctttactcctgtgtgaatcccctgatgtacaatgagctgtgacttgaatgtaaaggcttttccacaatcactacaaacataaggtttctcccctgtatgggttctctgatgtaccataaggtttgactttgtattaaaggctttctgacattcattgcattcatatggtttctctcctgtatgaattctttcatgtataatgagctgtgattttaaaccaaaagctttcccacattcattacacacatatggtttctgtcctgaatgagttttctggtgtgaaacaagctggtctttcctactgaagactttcccacattcacagcactcatagggattctcacctgtgtgaattctctgatgtataacaagctgtgaatggaaactgaatgttttcctgcattcactgcattcatgtagtttctctcctgtatgaattctctgatgtacaatgaggtatgatttactactgaagtctttcccacattcattacaaccatagggtttctcttcggcatgagtttgctgatgcactagaaggtatgacttgctgctgaaggctttctcacaacagctgcatccaaagggtttttcgcccatatacatttgttggcacataagttgcgatttcttattgacggtttttccagattcaatactttcacagtattttattccaataacagtttgctcatgtttagaatggaagaatgattttccatgtacctgaaacccattaggattatttctagcataatcactagtgaaatctatatatttcaaactctttccatgcgtgccacatttatgaggtttttgtcttgaaagatactttgtactaagaagacatagttttccaaatgtagtgcattcaaagctttttgccgtacttcccagcttgtctttattttcctgatgccaatccataagatcatcaattttccagactgtgtctccagaggatgcagcaacaaggcgtcatcttggaagcacagagcaggccctcaccagacaccaaacctgccagcaccttggctttggactttccagccttcaaaattggacaggtctgatttggaacttgggcctgcaccatacacagctcttctccttgttccaacttgaagatgatatcaggtttggtgtgttggtaccctagggacaccaggttgctatagttctccaacatcacactcctgtacaggcacttctgtgctgggtctagcagctgccactcctcccaggtaaaatccacaaacacatccatgaatgacaaaggtccccaggacttggtgatttttggctgctcttgggaaataaacagccactctaggactttctctattctgcgactcttctgcttctgcctgggtgttccagggagaggttgcagaccaggagtcccttggcccaagatggattcctgaccttggagctttctgatcctatcccatgaactgtttcgttcttggagaggtgggacccaaatagaagctgtccggaccctggtggccatccctacggtcagttttgtgtgcctcgctggaagtgacaggacgcgagggatgctccggctcctccaaaccctgaaggggcagcagaatagagtccagggtactgcctccacctccagatctgcagccagaagggttcgcaaccactccagactcggctggcccgttgaccacgacgggcgatgaacgctatctgaggaacaaggatctcgccatcggcgcggaacaatggcggccgctacgtat

SEQ ID NO: 18792 - RNA, 12350 nt, Homo sapiens
  source 1..12350: mol_type = other RNA
tgatatgtttgatattgggttgtctttttgttgttgggttgtaagagttctttatatgttctggatactagacccttatcaggtatattattttacagtgtcttttctcctatattcaccttttttttttttgagacggagtctcgctctgtcgcccaggctggagtgcagtggtgagatctgggctcactggttccaggttcacgccattctccttcctcagcctcccaagtagctgggactacaggcttccactaccagcctggctaattttttgtatttttttgtagagacagggtttcaccacattagccaggatggtttcgatctcctgacctcgtgatccacctgcctcagcctcccaaagtgctaggattacaggcgtgagccaccacacccggccttttttttttttttgagatggaattttgctttcttgctctgtcacctgggctggagtgcagtagcatgatctcggctcactgcaacctccacctcacagcttcaagcgatcctcctgcctcagcttcctgagttgctgggattacaggcacatgccaccacacccggcttttttttttctctttttttttatttttagtagagacgtggtttcaccaagttaaccaggctggtctcgcactcctgacctcaagtgatcctcccaccttggcctcccaaagtgctggaattacaggcgtgagccaccacacccagctccttttcactttcttgatagtgtccactgatgccgaaagttttcaattttggtgaagtccaatttacctattttttcttttgtttcccatgcttctggtgtcatatccaataaatcattgccaaatccagtgccaagaagtacatgaaaagattttcaacatcactagccattaggtaaaggaaaatcaaaaccacaatgagataccatttcatacatgttagagtggctattataaaaaatatggaggccaagtgcagtggttcaagcctgtaatcccagcactttgggaggccaaggtaagtggatcacttgaggacaggagtttgagactagcctggcctggccaacatggtgaaaccctgtctctactaaaaatacaaaaaatagccatacatggtggcacatgcctgtaatcccagctactcaggaggccgaggaaggagaatcacttaaacctaggaggcggaggttgcagtgagctgaaatggtgccactgcactccagcctgggtgacagagtgaaactccatttcaaaaaaaccaaaaaactatttgggtgtagtggcacctgtagttccagctacccaggaggctgaggtggaaggatcccttgagcccaggaggttggggctgcagtgagttatgatcatgcctatgaaatgagagagaaacaaactaattaatattggcaagtatgtggagaaattggaagccttgtgcactgctggtggaatgtaaaatgatagttgcacaataatggaaataatgtacttcatgccactgaagtgtacacttaaaaatagttaaaatggtaaatgttcttattatatatatgtgtatatatatgtgtatatgtgtatatatatgtgtatatatgtgtgtatgtgtgtgtgtatatatacatatatatatatatatatatatatatatatatatatatatatatatatatataaaatcacacatgaaagtctcccttggaactgatcctgaaataatttcatgtgtgatgaaagaacaccctgctctcctggagtgataagtggcctttttgttcatgctggcattatacatcccaggctcttccacacacacccagcataatttcaccaagcagagggagtacactctccaaaggcccatttgtgcctgtttctatcattatatcctcctatttaactcactccctgccctctacaaaccgtcatcaatcacagatatgtttgctacccctgtagtttctgcttttccataacatcatagaaataggatcatacagccttttcacactggtctctttcacttagcaatatgcctatcagattcatccatgtcctgcatggcctcagagcttgctcttgctgaacaggactccattgcatggatgtaccccagcctagttagtcattcacctattgaaggttatcctgattccttaaagtatttgtctgttatgaaaagagctgctgtacgtgagtacatgctgggttttgtttagatcaaactcctatgttttcaaagcagttatctaaatacctaggagtgtgattgttggctcatattgtgaagctttgtttagctttggggaaaagtcaaactatcttccaaagtggctatactattatgcattgcaccagcaatgaatgagagttcctgttgcaattgcaaatttacttatttttagattatagtcactttaatagatgtgcggtgctatctcgttgttttaatttgcttttccctcatgacaagtgtcactgagcattatttggtatgcttatttgccatctgtatatcttcttttttttttttttgagacggagtttcactcttgttgcccaggctggagtgcaatggcgcgatctcggctcacagcaacctccgcctcccgggttcaagccattctcctgcctccgcctccggagtagctaccacttggtggcagagtagcgccaccacgcctggctaattttgtatttttagtagagacagggtttctccatgttggtcaggctggtctcgaactccggacctcaggtgatctgcccgcctcggcctcccaaagtgctgggattacaggcgtgagccaccgtgcctggccaccatctgtatatctttggaaagtatgtatttggatctgtccccatttttaattgggttgtcttcttgttcaattttagggttttttttttatattttgcatacaaacactttttcagatttttttgaatgattttattcattacaaattccaattattgctatacattatttcaaatatataggaaatcacttgacttttgtctatggccatctactttgccttttattatctctatccattccaattaaggcatggaatgatggactctatttcagtttcgttttccaaaattatggcatggaaaatcgtaagattgaatttcaggggttcactgggactgcaagagggggcacatggccatcacaaaacaggaagcactgaccatccaacactgtgcctaggtagtaaggaaggggtgcaagcacacaccttgtctagcctgcttgcagtacctgcattctgctcacagacctctgggttgaatccacagaggaccaggccttccttctactcaggacctggggatcactagaggctgcatcacagtaaagactgagctgccttctcctcaggactgacctggggacccttggcaggggggaatccacagtgacaaacagaccttgcttctactcaggacccggagacccccgagggcacttcacagtgatgaccagaatttacctcatctcaggaccaacctgggggatgcatcacactgagaaccagagcttccttctccactggccaacctgaggaccactgtggggcacaaccacagtgaagactggagcttgtttctcttcaggactgacctagggaccctagtggggcaaatccacagtgaggttctgagcttccttctcctcaggaccaacctggggacccctgggaggtagatcacagtgatgaccagagtatcctcctcaggactgacccgtggtgggggatgcaaccacagtgaggactaaagcttccttttcctcacaacctggggaccccctagggggatacatcacagtgagatccagagcttccatatctgaagactcctgtagggtacacccacagtgacgaccagtgcactttccggaccaatctggggcgatgtcatctcacctttgggatacatggaggccacaggaggaaaagatgaggaaaagtgaggcctgcaccctgagtgctgaggagggagctttgctgtttcactttgccctgtaatatctgaacaagatttattttaggaaatcgtacctctattgaggtttccactagtcatctttatagcaagcccaactactttttatacatatgggtttgtttctggggagaaatcccagtacaaaaaaagggagaaacactgcgacaaaacactgcaacagtccaggtcaaagttggggatgaacagcacctgtgggatcaccctggatcccaagagggaagggcaaatgtgcaccctatgtgcttgcttttattaattttttttgaaggagtctcactctgctgcccgggctggagtgcaatggcacaatctcagctcactgcaacctccgcctctccagttcaagcaattctcctgagtagcttggattatagatgcatgccaccacagctggccaatttttgtatttttagtagagacggggtttcaccaggctggtctcgaactcctgacctcaagtcatccacctgcctcagcctcacaaaatgctgagattacaggcatgagccaccatgcccagcctttttattaatgttttaatggcctgtgtttctaacaagtagttgaaacaatgttgaaaattaaagagtagacatgttaaaacttgcaacttcatttaaatttaaatatatcatttataccaaaatcagaatttatttaagatttatggctgggtgcttggctcacacctgtaatcctagcactttgggaggccaaggcaggtggactgcttgagcccaggagtttgaaaccagactggaaaacatggtaaaaccccatctctacaagaaataaataactctacctggccctttagcaaagaattaagaaaaatcaatacagaccagtggctcacacctgtaatcccagcactttgggaggctgagggtggatcacgaggtcaggagttcaagaccagcctggccaacatggtgaaaccccatctctactaaaaacacaaaaattagctgggcgtggtggcgtgtgcctgtaattccagctactagggaggctgaggcaggagaattgcttgaacccaggaggcagaggttgcagtgagccaagaacacaccactgcactccagcctggcaatacagcgagactccatctcaaaaaaaaaaaaaaaaatgcaaatactatgccatataaggagcttgagcatccacagggagtatctgtggttgcgggggggtcctccatgaatactgacaactgcatacttgctactctactggcagttccaaacatttgtttgtggtttattttgggtttcctaattacacgatcacatctccaattcatggcagttgtttctgcacccatccctaattcctcacattccttgttttcacaccttggctagatgttactcatttcataaaagtgatgcgcattcttgtaattttgctttgttttttacagacagggtctcactttgttgcccaggatggagtgcaggggcatgatcatagctcactgtagccttgaactactggactcaagctaacctcctgcctcagcctcctcagtaggtgggactaccggcacttgccactacacctggctgatcttttttttgagatggaggcttgttctgtcgcccagcctggagtgcagtggtgcaatcttggctcactgcaactgccacctcctaggttcaagcaattcttctgcctcagcctcccgagtagatgggattacaggcacgtgccaccacacctggctgacttttgtatttttagtagagacggggtttcaccatgttagccacactggtcttgaaatcctgacctcaagtgatctgcccacctcggcctcccaaagtgctgggattacaggcatgagccacggcgcctgaccacacctggctaatctttttaaaaagtttttgtacagacagggtctccctatattggtcaggcttgtctcgaactcctgggttccagcaatcctccagcctcagccttcccaagtgctggtattacatggatgagccactgcacctggctaattttactttaaaggaatctttctactattttatcattaagtatgacatttgtgttttcagaacatatattccctaccaagttacaggagttaattttaattcccaacttaatagtattttagtgtcatctatgggtgttaaattccatcaagtgatttatcagcatatactgagataatccttatgagttttatctggtagttaattaaaatattttctaatattaaatcttccaaacatactcttctgttttttgagacagggtctagttctgtcacccagggtggagtacagtggtacgatctcagctcactgcaacttccgcctcctagattcaagtgattctcccgtcccagcctcccaagtagctgggattataggtgtcagttaccatgccctgctatttttttgtatttttagtagagaggggtttcaccatgttggccaggctggtctcaaactcctgacctcaggtgatccaccatctcagcctcctgaagtgctgggattataggtgtgagccaccgtgcctggccccatatatctctttttaagtgggcatactgccattataaataatagtgattctgctggtaatgaacaaaggatgctggatccactaatagtctgttaaacctaatatcatgactttcttgttagctatacattggtttgctataattccatttagaatttttaaacctatgttcacaaatatggatttttaaacctatgttcacaaatatggatttttaaacctatgttcacaaatatggtttgcaagtcattttttctcctaaatttctatttgatggggaagttgtaaaatattggggttatttttccttggattttccttataataactattcctgaaaagtctctggaatgtctttcttttctggggctggggtagaaggactagatagatttacaaaccagtaactcaatttctgttttgtaaaattttcatttcattaaataataagtcctaatcaagtattattctttcccacagtatgtgagtgctgtcctcaatactgtcaacacttctggcttctaccaggcaaggctgcatgtagatttgcatctgaaaaaacaacaaactaaaatctaaccctaggtagtagtaaactgaatataaactttctcttatgaatttattctgtcttctttggtacatcaataataatatacacctttacagtatttcccagattgggggatacactttagcaagtatctgcgattatttgtttatgtaagatgtcccttcccttctgtgaatcatcattcttcaccccaagtatcttgagattggattctgtataagcagaatacaacagttaggcattcaggtatcattaaattcctccgcttcaaggatgaaaatttctttgggtatctaatagagtacaaagcagaaggtgtttcagaaatatttgcagtattgaatccgcatattcctccaagatagccctaatctaactggcagggtcccactcttcccagattaatgcccactcacataacaaacctgatgaggtagtgaagaaaactaactttgtgagtaagcaactggcagagtttttcaccactgtgactctatagctacatgtaactaagtagtatcactgacacataatcttaaattgaagttttaagatcattattctccatgttatacatgggtatcaaaagcattcccctcttgaccactccagaattctgtttaaaatttttcaatgacaacttatccatttccccaaagcctcagtgagcacatgatgccaacaattcatttcatgacttcatagcatgggccaagtttcttgcttaaaagacttccatcctgtcttgggaaacaaccatttccaaatatccacatatccttgcaagtttctgcctactcctctaccacccatttctgaagccatctgatttagtaagctgtatgcaaaagatacacaatggctaatgcaatcaaacaaggaatgtattaaaagcacacccaatagctcaaaataaaagacaagtgaacaaagttaagaaaatgacagtaacaaaagctgttctgggaacctctattgaaatagctacttattacatcaacatgctaccacagaacaaaagctcatgttgcttttctgaacttgaaaaacccattaacaatgtacagttctgagcctcagctgaccatagtgctcatgccaagtcctgagcagggcatcttgaatggtggttccctcatgactacatacaccgttagggaatgtttcgttaagaggaaatcaagatgttctaacctgtgaaggtagaatagattccaggctacacaaacacatgaagtgtgccttatattgattactaaagaggttgctgccaagactgcttccaaagggcagaagatagccctaaaaaatgtttgcagtgtggaaatgcatttttagtaagtcatattctagtaacaagttgcatttggtaagacacaaagaaacaatgttggtatgcagagtagaaatctctggaagatgatattgtcatatcagagatattgtcagtatcagagatactgaaatctctggaagatgatttttgtctcacatatggcattcgcaagtaaaatgccaaactgcaaaattcatattatgtagtacacataggaagatatctaaatatccctgtaggctctgggatgttatttcttattcttaacctccttactagattcacttgtacaatgaaataatctgtatcttattatttataattgagaattttctcaaaccttttcctgaaattttggaacacctggaataaaatttcttaaaatgattcctaaaagaaataattcttcaaaattaatattaagatataataacaggttggtttttttttttttttttttttttttttttagaatgaagcttctaaggtgaggttaacagtccagctgtggtttatttggtacattcataagatgttcactcctatatatattttttccctaggggtttctcatttctagatttacactttcccttatagcatggtccctccaaggtatatgcttccgatacataaaatgtttgtaattttgttaattctgccattcattagctcaataatttctctcattaaaattctgtaaactatgaatttcaaagaagtctattctatattcatctggttcatgaagtttcctctttgtgaatcttattttagtaaaatgactttacaacgtttaacatggttcctcacctgtatgaactttttaaaaaaaggtatgacttgctgctaaaaattttcagagtggttactaaattcagttttcctgtgtattgtctactatctttttgcatgtaaagaacagctttctgtggatgcctttccatatgctgtgcattcataaagtttctattcagtatgagttttctggaagatgacaagatgattccacttacagagtttctctttatatatgattgtttctatctcttgtgaatccacttttcagagtttcgtaaaattatcaatgtttgtcatctacatgagttctctgatgcataatgagctgtgacttccaacaaaaggctttcccacattcagtgcacttacaaggcttctctcctgtatgtgttctctgatgtgcactgagaattgatttttgagagaaggttttcccacattcattgcacccatagggtttctctcctgaatgagttctttgatgtacaatgagttgagaattcctaatgaaggcttttccacactcactgcattcatatggtttctctcttgtgtgcattctctggtgtacaagaaggcgtaatttcccactgaaggatttctcacattgactgcatttataagggttgacccctgcatgagttcgctcatgtacaatgagtagtgatttccaaatgaaggctttcccacattcattacattcatatggtttttcacctgaatgagttctcatgtgtataattaggtatgacttgctgctaaaagctttcccacattcactgcacccataaggcttttcccctgcatgagttcgctgatgtgaaatgagctggtctttcctattaaaggctttcccacattcactgcattcatagggattttctcctgtgtgaattctctgatgcacaatgagttgtgaattgaaactaaaggatttcccgcattccctgcactcatgtggtttctctcctgtatgagttctcatatgtataataaggtatgacttgctcctgaaggctttcccacactcactgcatccatatggttttactcctgtgtgacttctctgatgtacaatgagctgggacttcaaactaaaggtttttgcacattgactgcatccatagggttttactccagtgtgcactcctttatgtacaatgagctgtgatttgaacgtaaaggcttttccacattcattacaactatagggtttctctcctgtatgagttctctgatgtacaatcaggtttgactttgtattaaaggctttctgacactcactacattcaaatggtttctcccctgtatgagttctctggtgtataataagctgtgactttaaaccaaaagcctttccacagtcggtgcattcataaggcttctctcctgcatgagttctctggtgtgaaataagctggtatttccgactgaaggctttcccacattcatggcattcataggggttctctcctgtatgaatcctctgatgtataatgagctgtgatttaaaactgaaggctttcccacaattgttgcattcatggagtttttctcctgtatgagtccttgtatgtataataaggtatgacttgctcctgaaggctttgccacattcattgcatacataaggtttcattcctgtgtgacttctctgatgtacaatgagctgtgatttcaaactgaatcctttaccacactgaatacacccatagggctttactcctgtgtgaatcccctgatgtacaatgagctgtgacttgaatgtaaaggcttttccacaatcactacaaacataaggtttctcccctgtatgggttctctgatgtaccataaggtttgactttgtattaaaggctttctgacattcattgcattcatatggtttctctcctgtatgaattctttcatgtataatgagctgtgattttaaaccaaaagctttcccacattcattacacacatatggtttctgtcctgaatgagttttctggtgtgaaacaagctggtctttcctactgaagactttcccacattcacagcactcatagggattctcacctgtgtgaattctctgatgtataacaagctgtgaatggaaactgaatgttttcctgcattcactgcattcatgtagtttctctcctgtatgaattctctgatgtacaatgaggtatgatttactactgaagtctttcccacattcattacaaccatagggtttctcttcggcatgagtttgctgatgcactagaaggtatgacttgctgctgaaggctttctcacaacagctgcatccaaagggtttttcgcccatatacatttgttggcacataagttgcgatttcttattgacggtttttccagattcaatactttcacagtattttattccaataacagtttgctcatgtttagaatggaagaatgattttccatgtacctgaaacccattaggattatttctagcataatcactagtgaaatctatatatttcaaactctttccatgcgtgccacatttatgaggtttttgtcttgaaagatactttgtactaagaagacatagttttccaaatgtagtgcattcaaagctttttgccgtacttcccagcttgtctttattttcctgatgccaatccataagatcatcaattttccagactgtgtttggacaggtctgatttggaacttgggcctgcaccatacacagctcttctccttgttccaacttgaagatgatatcaggtttggtgtgttggtaccccaaatagaagctgtccggaccctggtggccatccctacggtcagttttgtgtgcctcgctggaagtgacaggacgcgagggatgctccggctcctccaaaccctgaaggggcagcagaatagagtccagggtactgcctccacctccagatctgcagccagaagggttcgcaaccactccagactcggctggcccgttgaccacgacgggcgatgaacgctatctgaggaacaaggatctcgccatcggcgcggaacaatggcggccgctacgtat

SEQ ID NO: 18793 - RNA, 12551 nt, Homo sapiens
  source 1..12551: mol_type = other RNA
tgatatgtttgatattgggttgtctttttgttgttgggttgtaagagttctttatatgttctggatactagacccttatcaggtatattattttacagtgtcttttctcctatattcaccttttttttttttgagacggagtctcgctctgtcgcccaggctggagtgcagtggtgagatctgggctcactggttccaggttcacgccattctccttcctcagcctcccaagtagctgggactacaggcttccactaccagcctggctaattttttgtatttttttgtagagacagggtttcaccacattagccaggatggtttcgatctcctgacctcgtgatccacctgcctcagcctcccaaagtgctaggattacaggcgtgagccaccacacccggccttttttttttttttgagatggaattttgctttcttgctctgtcacctgggctggagtgcagtagcatgatctcggctcactgcaacctccacctcacagcttcaagcgatcctcctgcctcagcttcctgagttgctgggattacaggcacatgccaccacacccggcttttttttttctctttttttttatttttagtagagacgtggtttcaccaagttaaccaggctggtctcgcactcctgacctcaagtgatcctcccaccttggcctcccaaagtgctggaattacaggcgtgagccaccacacccagctccttttcactttcttgatagtgtccactgatgccgaaagttttcaattttggtgaagtccaatttacctattttttcttttgtttcccatgcttctggtgtcatatccaataaatcattgccaaatccagtgccaagaagtacatgaaaagattttcaacatcactagccattaggtaaaggaaaatcaaaaccacaatgagataccatttcatacatgttagagtggctattataaaaaatatggaggccaagtgcagtggttcaagcctgtaatcccagcactttgggaggccaaggtaagtggatcacttgaggacaggagtttgagactagcctggcctggccaacatggtgaaaccctgtctctactaaaaatacaaaaaatagccatacatggtggcacatgcctgtaatcccagctactcaggaggccgaggaaggagaatcacttaaacctaggaggcggaggttgcagtgagctgaaatggtgccactgcactccagcctgggtgacagagtgaaactccatttcaaaaaaaccaaaaaactatttgggtgtagtggcacctgtagttccagctacccaggaggctgaggtggaaggatcccttgagcccaggaggttggggctgcagtgagttatgatcatgcctatgaaatgagagagaaacaaactaattaatattggcaagtatgtggagaaattggaagccttgtgcactgctggtggaatgtaaaatgatagttgcacaataatggaaataatgtacttcatgccactgaagtgtacacttaaaaatagttaaaatggtaaatgttcttattatatatatgtgtatatatatgtgtatatgtgtatatatatgtgtatatatgtgtgtatgtgtgtgtgtatatatacatatatatatatatatatatatatatatatatatatatatatatatatatataaaatcacacatgaaagtctcccttggaactgatcctgaaataatttcatgtgtgatgaaagaacaccctgctctcctggagtgataagtggcctttttgttcatgctggcattatacatcccaggctcttccacacacacccagcataatttcaccaagcagagggagtacactctccaaaggcccatttgtgcctgtttctatcattatatcctcctatttaactcactccctgccctctacaaaccgtcatcaatcacagatatgtttgctacccctgtagtttctgcttttccataacatcatagaaataggatcatacagccttttcacactggtctctttcacttagcaatatgcctatcagattcatccatgtcctgcatggcctcagagcttgctcttgctgaacaggactccattgcatggatgtaccccagcctagttagtcattcacctattgaaggttatcctgattccttaaagtatttgtctgttatgaaaagagctgctgtacgtgagtacatgctgggttttgtttagatcaaactcctatgttttcaaagcagttatctaaatacctaggagtgtgattgttggctcatattgtgaagctttgtttagctttggggaaaagtcaaactatcttccaaagtggctatactattatgcattgcaccagcaatgaatgagagttcctgttgcaattgcaaatttacttatttttagattatagtcactttaatagatgtgcggtgctatctcgttgttttaatttgcttttccctcatgacaagtgtcactgagcattatttggtatgcttatttgccatctgtatatcttcttttttttttttttgagacggagtttcactcttgttgcccaggctggagtgcaatggcgcgatctcggctcacagcaacctccgcctcccgggttcaagccattctcctgcctccgcctccggagtagctaccacttggtggcagagtagcgccaccacgcctggctaattttgtatttttagtagagacagggtttctccatgttggtcaggctggtctcgaactccggacctcaggtgatctgcccgcctcggcctcccaaagtgctgggattacaggcgtgagccaccgtgcctggccaccatctgtatatctttggaaagtatgtatttggatctgtccccatttttaattgggttgtcttcttgttcaattttagggttttttttttatattttgcatacaaacactttttcagatttttttgaatgattttattcattacaaattccaattattgctatacattatttcaaatatataggaaatcacttgacttttgtctatggccatctactttgccttttattatctctatccattccaattaaggcatggaatgatggactctatttcagtttcgttttccaaaattatggcatggaaaatcgtaagattgaatttcaggggttcactgggactgcaagagggggcacatggccatcacaaaacaggaagcactgaccatccaacactgtgcctaggtagtaaggaaggggtgcaagcacacaccttgtctagcctgcttgcagtacctgcattctgctcacagacctctgggttgaatccacagaggaccaggccttccttctactcaggacctggggatcactagaggctgcatcacagtaaagactgagctgccttctcctcaggactgacctggggacccttggcaggggggaatccacagtgacaaacagaccttgcttctactcaggacccggagacccccgagggcacttcacagtgatgaccagaatttacctcatctcaggaccaacctgggggatgcatcacactgagaaccagagcttccttctccactggccaacctgaggaccactgtggggcacaaccacagtgaagactggagcttgtttctcttcaggactgacctagggaccctagtggggcaaatccacagtgaggttctgagcttccttctcctcaggaccaacctggggacccctgggaggtagatcacagtgatgaccagagtatcctcctcaggactgacccgtggtgggggatgcaaccacagtgaggactaaagcttccttttcctcacaacctggggaccccctagggggatacatcacagtgagatccagagcttccatatctgaagactcctgtagggtacacccacagtgacgaccagtgcactttccggaccaatctggggcgatgtcatctcacctttgggatacatggaggccacaggaggaaaagatgaggaaaagtgaggcctgcaccctgagtgctgaggagggagctttgctgtttcactttgccctgtaatatctgaacaagatttattttaggaaatcgtacctctattgaggtttccactagtcatctttatagcaagcccaactactttttatacatatgggtttgtttctggggagaaatcccagtacaaaaaaagggagaaacactgcgacaaaacactgcaacagtccaggtcaaagttggggatgaacagcacctgtgggatcaccctggatcccaagagggaagggcaaatgtgcaccctatgtgcttgcttttattaattttttttgaaggagtctcactctgctgcccgggctggagtgcaatggcacaatctcagctcactgcaacctccgcctctccagttcaagcaattctcctgagtagcttggattatagatgcatgccaccacagctggccaatttttgtatttttagtagagacggggtttcaccaggctggtctcgaactcctgacctcaagtcatccacctgcctcagcctcacaaaatgctgagattacaggcatgagccaccatgcccagcctttttattaatgttttaatggcctgtgtttctaacaagtagttgaaacaatgttgaaaattaaagagtagacatgttaaaacttgcaacttcatttaaatttaaatatatcatttataccaaaatcagaatttatttaagatttatggctgggtgcttggctcacacctgtaatcctagcactttgggaggccaaggcaggtggactgcttgagcccaggagtttgaaaccagactggaaaacatggtaaaaccccatctctacaagaaataaataactctacctggccctttagcaaagaattaagaaaaatcaatacagaccagtggctcacacctgtaatcccagcactttgggaggctgagggtggatcacgaggtcaggagttcaagaccagcctggccaacatggtgaaaccccatctctactaaaaacacaaaaattagctgggcgtggtggcgtgtgcctgtaattccagctactagggaggctgaggcaggagaattgcttgaacccaggaggcagaggttgcagtgagccaagaacacaccactgcactccagcctggcaatacagcgagactccatctcaaaaaaaaaaaaaaaaatgcaaatactatgccatataaggagcttgagcatccacagggagtatctgtggttgcgggggggtcctccatgaatactgacaactgcatacttgctactctactggcagttccaaacatttgtttgtggtttattttgggtttcctaattacacgatcacatctccaattcatggcagttgtttctgcacccatccctaattcctcacattccttgttttcacaccttggctagatgttactcatttcataaaagtgatgcgcattcttgtaattttgctttgttttttacagacagggtctcactttgttgcccaggatggagtgcaggggcatgatcatagctcactgtagccttgaactactggactcaagctaacctcctgcctcagcctcctcagtaggtgggactaccggcacttgccactacacctggctgatcttttttttgagatggaggcttgttctgtcgcccagcctggagtgcagtggtgcaatcttggctcactgcaactgccacctcctaggttcaagcaattcttctgcctcagcctcccgagtagatgggattacaggcacgtgccaccacacctggctgacttttgtatttttagtagagacggggtttcaccatgttagccacactggtcttgaaatcctgacctcaagtgatctgcccacctcggcctcccaaagtgctgggattacaggcatgagccacggcgcctgaccacacctggctaatctttttaaaaagtttttgtacagacagggtctccctatattggtcaggcttgtctcgaactcctgggttccagcaatcctccagcctcagccttcccaagtgctggtattacatggatgagccactgcacctggctaattttactttaaaggaatctttctactattttatcattaagtatgacatttgtgttttcagaacatatattccctaccaagttacaggagttaattttaattcccaacttaatagtattttagtgtcatctatgggtgttaaattccatcaagtgatttatcagcatatactgagataatccttatgagttttatctggtagttaattaaaatattttctaatattaaatcttccaaacatactcttctgttttttgagacagggtctagttctgtcacccagggtggagtacagtggtacgatctcagctcactgcaacttccgcctcctagattcaagtgattctcccgtcccagcctcccaagtagctgggattataggtgtcagttaccatgccctgctatttttttgtatttttagtagagaggggtttcaccatgttggccaggctggtctcaaactcctgacctcaggtgatccaccatctcagcctcctgaagtgctgggattataggtgtgagccaccgtgcctggccccatatatctctttttaagtgggcatactgccattataaataatagtgattctgctggtaatgaacaaaggatgctggatccactaatagtctgttaaacctaatatcatgactttcttgttagctatacattggtttgctataattccatttagaatttttaaacctatgttcacaaatatggatttttaaacctatgttcacaaatatggatttttaaacctatgttcacaaatatggtttgcaagtcattttttctcctaaatttctatttgatggggaagttgtaaaatattggggttatttttccttggattttccttataataactattcctgaaaagtctctggaatgtctttcttttctggggctggggtagaaggactagatagatttacaaaccagtaactcaatttctgttttgtaaaattttcatttcattaaataataagtcctaatcaagtattattctttcccacagtatgtgagtgctgtcctcaatactgtcaacacttctggcttctaccaggcaaggctgcatgtagatttgcatctgaaaaaacaacaaactaaaatctaaccctaggtagtagtaaactgaatataaactttctcttatgaatttattctgtcttctttggtacatcaataataatatacacctttacagtatttcccagattgggggatacactttagcaagtatctgcgattatttgtttatgtaagatgtcccttcccttctgtgaatcatcattcttcaccccaagtatcttgagattggattctgtataagcagaatacaacagttaggcattcaggtatcattaaattcctccgcttcaaggatgaaaatttctttgggtatctaatagagtacaaagcagaaggtgtttcagaaatatttgcagtattgaatccgcatattcctccaagatagccctaatctaactggcagggtcccactcttcccagattaatgcccactcacataacaaacctgatgaggtagtgaagaaaactaactttgtgagtaagcaactggcagagtttttcaccactgtgactctatagctacatgtaactaagtagtatcactgacacataatcttaaattgaagttttaagatcattattctccatgttatacatgggtatcaaaagcattcccctcttgaccactccagaattctgtttaaaatttttcaatgacaacttatccatttccccaaagcctcagtgagcacatgatgccaacaattcatttcatgacttcatagcatgggccaagtttcttgcttaaaagacttccatcctgtcttgggaaacaaccatttccaaatatccacatatccttgcaagtttctgcctactcctctaccacccatttctgaagccatctgatttagtaagctgtatgcaaaagatacacaatggctaatgcaatcaaacaaggaatgtattaaaagcacacccaatagctcaaaataaaagacaagtgaacaaagttaagaaaatgacagtaacaaaagctgttctgggaacctctattgaaatagctacttattacatcaacatgctaccacagaacaaaagctcatgttgcttttctgaacttgaaaaacccattaacaatgtacagttctgagcctcagctgaccatagtgctcatgccaagtcctgagcagggcatcttgaatggtggttccctcatgactacatacaccgttagggaatgtttcgttaagaggaaatcaagatgttctaacctgtgaaggtagaatagattccaggctacacaaacacatgaagtgtgccttatattgattactaaagaggttgctgccaagactgcttccaaagggcagaagatagccctaaaaaatgtttgcagtgtggaaatgcatttttagtaagtcatattctagtaacaagttgcatttggtaagacacaaagaaacaatgttggtatgcagagtagaaatctctggaagatgatattgtcatatcagagatattgtcagtatcagagatactgaaatctctggaagatgatttttgtctcacatatggcattcgcaagtaaaatgccaaactgcaaaattcatattatgtagtacacataggaagatatctaaatatccctgtaggctctgggatgttatttcttattcttaacctccttactagattcacttgtacaatgaaataatctgtatcttattatttataattgagaattttctcaaaccttttcctgaaattttggaacacctggaataaaatttcttaaaatgattcctaaaagaaataattcttcaaaattaatattaagatataataacaggttggtttttttttttttttttttttttttttttagaatgaagcttctaaggtgaggttaacagtccagctgtggtttatttggtacattcataagatgttcactcctatatatattttttccctaggggtttctcatttctagatttacactttcccttatagcatggtccctccaaggtatatgcttccgatacataaaatgtttgtaattttgttaattctgccattcattagctcaataatttctctcattaaaattctgtaaactatgaatttcaaagaagtctattctatattcatctggttcatgaagtttcctctttgtgaatcttattttagtaaaatgactttacaacgtttaacatggttcctcacctgtatgaactttttaaaaaaaggtatgacttgctgctaaaaattttcagagtggttactaaattcagttttcctgtgtattgtctactatctttttgcatgtaaagaacagctttctgtggatgcctttccatatgctgtgcattcataaagtttctattcagtatgagttttctggaagatgacaagatgattccacttacagagtttctctttatatatgattgtttctatctcttgtgaatccacttttcagagtttcgtaaaattatcaatgtttgtcatctacatgagttctctgatgcataatgagctgtgacttccaacaaaaggctttcccacattcagtgcacttacaaggcttctctcctgtatgtgttctctgatgtgcactgagaattgatttttgagagaaggttttcccacattcattgcacccatagggtttctctcctgaatgagttctttgatgtacaatgagttgagaattcctaatgaaggcttttccacactcactgcattcatatggtttctctcttgtgtgcattctctggtgtacaagaaggcgtaatttcccactgaaggatttctcacattgactgcatttataagggttgacccctgcatgagttcgctcatgtacaatgagtagtgatttccaaatgaaggctttcccacattcattacattcatatggtttttcacctgaatgagttctcatgtgtataattaggtatgacttgctgctaaaagctttcccacattcactgcacccataaggcttttcccctgcatgagttcgctgatgtgaaatgagctggtctttcctattaaaggctttcccacattcactgcattcatagggattttctcctgtgtgaattctctgatgcacaatgagttgtgaattgaaactaaaggatttcccgcattccctgcactcatgtggtttctctcctgtatgagttctcatatgtataataaggtatgacttgctcctgaaggctttcccacactcactgcatccatatggttttactcctgtgtgacttctctgatgtacaatgagctgggacttcaaactaaaggtttttgcacattgactgcatccatagggttttactccagtgtgcactcctttatgtacaatgagctgtgatttgaacgtaaaggcttttccacattcattacaactatagggtttctctcctgtatgagttctctgatgtacaatcaggtttgactttgtattaaaggctttctgacactcactacattcaaatggtttctcccctgtatgagttctctggtgtataataagctgtgactttaaaccaaaagcctttccacagtcggtgcattcataaggcttctctcctgcatgagttctctggtgtgaaataagctggtatttccgactgaaggctttcccacattcatggcattcataggggttctctcctgtatgaatcctctgatgtataatgagctgtgatttaaaactgaaggctttcccacaattgttgcattcatggagtttttctcctgtatgagtccttgtatgtataataaggtatgacttgctcctgaaggctttgccacattcattgcatacataaggtttcattcctgtgtgacttctctgatgtacaatgagctgtgatttcaaactgaatcctttaccacactgaatacacccatagggctttactcctgtgtgaatcccctgatgtacaatgagctgtgacttgaatgtaaaggcttttccacaatcactacaaacataaggtttctcccctgtatgggttctctgatgtaccataaggtttgactttgtattaaaggctttctgacattcattgcattcatatggtttctctcctgtatgaattctttcatgtataatgagctgtgattttaaaccaaaagctttcccacattcattacacacatatggtttctgtcctgaatgagttttctggtgtgaaacaagctggtctttcctactgaagactttcccacattcacagcactcatagggattctcacctgtgtgaattctctgatgtataacaagctgtgaatggaaactgaatgttttcctgcattcactgcattcatgtagtttctctcctgtatgaattctctgatgtacaatgaggtatgatttactactgaagtctttcccacattcattacaaccatagggtttctcttcggcatgagtttgctgatgcactagaaggtatgacttgctgctgaaggctttctcacaacagctgcatccaaagggtttttcgcccatatacatttgttggcacataagttgcgatttcttattgacggtttttccagattcaatactttcacagtattttattccaataacagtttgctcatgtttagaatggaagaatgattttccatgtacctgaaacccattaggattatttctagcataatcactagtgaaatctatatatttcaaactctttccatgcgtgccacatttatgaggtttttgtcttgaaagatactttgtactaagaagacatagttttccaaatgtagtgcattcaaagctttttgccgtacttcccagcttgtctttattttcctgatgccaatccataagatcatcaattttccagactgtgtttggacaggtctgatttggaacttgggcctgcaccatacacagctcttctccttgttccaacttgaagatgatatcaggtttggtgtgttggtaccccaggacttggtgatttttggctgctcttgggaaataaacagccactctaggactttctctattctgcgactcttctgcttctgcctgggtgttccagggagaggttgcagaccaggagtcccttggcccaagatggattcctgaccttggagctttctgatcctatcccatgaactgtttcgttcttggagaggtgggacccaaatagaagctgtccggaccctggtggccatccctacggtcagttttgtgtgcctcgctggaagtgacaggacgcgagggatgctccggctcctccaaaccctgaaggggcagcagaatagagtccagggtactgcctccacctccagatctgcagccagaagggttcgcaaccactccagactcggctggcccgttgaccacgacgggcgatgaacgctatctgaggaacaaggatctcgccatcggcgcggaacaatggcggccgctacgtat

SEQ ID NO: 18794 - RNA, 12619 nt, Homo sapiens
  source 1..12619: mol_type = other RNA
tgatatgtttgatattgggttgtctttttgttgttgggttgtaagagttctttatatgttctggatactagacccttatcaggtatattattttacagtgtcttttctcctatattcaccttttttttttttgagacggagtctcgctctgtcgcccaggctggagtgcagtggtgagatctgggctcactggttccaggttcacgccattctccttcctcagcctcccaagtagctgggactacaggcttccactaccagcctggctaattttttgtatttttttgtagagacagggtttcaccacattagccaggatggtttcgatctcctgacctcgtgatccacctgcctcagcctcccaaagtgctaggattacaggcgtgagccaccacacccggccttttttttttttttgagatggaattttgctttcttgctctgtcacctgggctggagtgcagtagcatgatctcggctcactgcaacctccacctcacagcttcaagcgatcctcctgcctcagcttcctgagttgctgggattacaggcacatgccaccacacccggcttttttttttctctttttttttatttttagtagagacgtggtttcaccaagttaaccaggctggtctcgcactcctgacctcaagtgatcctcccaccttggcctcccaaagtgctggaattacaggcgtgagccaccacacccagctccttttcactttcttgatagtgtccactgatgccgaaagttttcaattttggtgaagtccaatttacctattttttcttttgtttcccatgcttctggtgtcatatccaataaatcattgccaaatccagtgccaagaagtacatgaaaagattttcaacatcactagccattaggtaaaggaaaatcaaaaccacaatgagataccatttcatacatgttagagtggctattataaaaaatatggaggccaagtgcagtggttcaagcctgtaatcccagcactttgggaggccaaggtaagtggatcacttgaggacaggagtttgagactagcctggcctggccaacatggtgaaaccctgtctctactaaaaatacaaaaaatagccatacatggtggcacatgcctgtaatcccagctactcaggaggccgaggaaggagaatcacttaaacctaggaggcggaggttgcagtgagctgaaatggtgccactgcactccagcctgggtgacagagtgaaactccatttcaaaaaaaccaaaaaactatttgggtgtagtggcacctgtagttccagctacccaggaggctgaggtggaaggatcccttgagcccaggaggttggggctgcagtgagttatgatcatgcctatgaaatgagagagaaacaaactaattaatattggcaagtatgtggagaaattggaagccttgtgcactgctggtggaatgtaaaatgatagttgcacaataatggaaataatgtacttcatgccactgaagtgtacacttaaaaatagttaaaatggtaaatgttcttattatatatatgtgtatatatatgtgtatatgtgtatatatatgtgtatatatgtgtgtatgtgtgtgtgtatatatacatatatatatatatatatatatatatatatatatatatatatatatatatataaaatcacacatgaaagtctcccttggaactgatcctgaaataatttcatgtgtgatgaaagaacaccctgctctcctggagtgataagtggcctttttgttcatgctggcattatacatcccaggctcttccacacacacccagcataatttcaccaagcagagggagtacactctccaaaggcccatttgtgcctgtttctatcattatatcctcctatttaactcactccctgccctctacaaaccgtcatcaatcacagatatgtttgctacccctgtagtttctgcttttccataacatcatagaaataggatcatacagccttttcacactggtctctttcacttagcaatatgcctatcagattcatccatgtcctgcatggcctcagagcttgctcttgctgaacaggactccattgcatggatgtaccccagcctagttagtcattcacctattgaaggttatcctgattccttaaagtatttgtctgttatgaaaagagctgctgtacgtgagtacatgctgggttttgtttagatcaaactcctatgttttcaaagcagttatctaaatacctaggagtgtgattgttggctcatattgtgaagctttgtttagctttggggaaaagtcaaactatcttccaaagtggctatactattatgcattgcaccagcaatgaatgagagttcctgttgcaattgcaaatttacttatttttagattatagtcactttaatagatgtgcggtgctatctcgttgttttaatttgcttttccctcatgacaagtgtcactgagcattatttggtatgcttatttgccatctgtatatcttcttttttttttttttgagacggagtttcactcttgttgcccaggctggagtgcaatggcgcgatctcggctcacagcaacctccgcctcccgggttcaagccattctcctgcctccgcctccggagtagctaccacttggtggcagagtagcgccaccacgcctggctaattttgtatttttagtagagacagggtttctccatgttggtcaggctggtctcgaactccggacctcaggtgatctgcccgcctcggcctcccaaagtgctgggattacaggcgtgagccaccgtgcctggccaccatctgtatatctttggaaagtatgtatttggatctgtccccatttttaattgggttgtcttcttgttcaattttagggttttttttttatattttgcatacaaacactttttcagatttttttgaatgattttattcattacaaattccaattattgctatacattatttcaaatatataggaaatcacttgacttttgtctatggccatctactttgccttttattatctctatccattccaattaaggcatggaatgatggactctatttcagtttcgttttccaaaattatggcatggaaaatcgtaagattgaatttcaggggttcactgggactgcaagagggggcacatggccatcacaaaacaggaagcactgaccatccaacactgtgcctaggtagtaaggaaggggtgcaagcacacaccttgtctagcctgcttgcagtacctgcattctgctcacagacctctgggttgaatccacagaggaccaggccttccttctactcaggacctggggatcactagaggctgcatcacagtaaagactgagctgccttctcctcaggactgacctggggacccttggcaggggggaatccacagtgacaaacagaccttgcttctactcaggacccggagacccccgagggcacttcacagtgatgaccagaatttacctcatctcaggaccaacctgggggatgcatcacactgagaaccagagcttccttctccactggccaacctgaggaccactgtggggcacaaccacagtgaagactggagcttgtttctcttcaggactgacctagggaccctagtggggcaaatccacagtgaggttctgagcttccttctcctcaggaccaacctggggacccctgggaggtagatcacagtgatgaccagagtatcctcctcaggactgacccgtggtgggggatgcaaccacagtgaggactaaagcttccttttcctcacaacctggggaccccctagggggatacatcacagtgagatccagagcttccatatctgaagactcctgtagggtacacccacagtgacgaccagtgcactttccggaccaatctggggcgatgtcatctcacctttgggatacatggaggccacaggaggaaaagatgaggaaaagtgaggcctgcaccctgagtgctgaggagggagctttgctgtttcactttgccctgtaatatctgaacaagatttattttaggaaatcgtacctctattgaggtttccactagtcatctttatagcaagcccaactactttttatacatatgggtttgtttctggggagaaatcccagtacaaaaaaagggagaaacactgcgacaaaacactgcaacagtccaggtcaaagttggggatgaacagcacctgtgggatcaccctggatcccaagagggaagggcaaatgtgcaccctatgtgcttgcttttattaattttttttgaaggagtctcactctgctgcccgggctggagtgcaatggcacaatctcagctcactgcaacctccgcctctccagttcaagcaattctcctgagtagcttggattatagatgcatgccaccacagctggccaatttttgtatttttagtagagacggggtttcaccaggctggtctcgaactcctgacctcaagtcatccacctgcctcagcctcacaaaatgctgagattacaggcatgagccaccatgcccagcctttttattaatgttttaatggcctgtgtttctaacaagtagttgaaacaatgttgaaaattaaagagtagacatgttaaaacttgcaacttcatttaaatttaaatatatcatttataccaaaatcagaatttatttaagatttatggctgggtgcttggctcacacctgtaatcctagcactttgggaggccaaggcaggtggactgcttgagcccaggagtttgaaaccagactggaaaacatggtaaaaccccatctctacaagaaataaataactctacctggccctttagcaaagaattaagaaaaatcaatacagaccagtggctcacacctgtaatcccagcactttgggaggctgagggtggatcacgaggtcaggagttcaagaccagcctggccaacatggtgaaaccccatctctactaaaaacacaaaaattagctgggcgtggtggcgtgtgcctgtaattccagctactagggaggctgaggcaggagaattgcttgaacccaggaggcagaggttgcagtgagccaagaacacaccactgcactccagcctggcaatacagcgagactccatctcaaaaaaaaaaaaaaaaatgcaaatactatgccatataaggagcttgagcatccacagggagtatctgtggttgcgggggggtcctccatgaatactgacaactgcatacttgctactctactggcagttccaaacatttgtttgtggtttattttgggtttcctaattacacgatcacatctccaattcatggcagttgtttctgcacccatccctaattcctcacattccttgttttcacaccttggctagatgttactcatttcataaaagtgatgcgcattcttgtaattttgctttgttttttacagacagggtctcactttgttgcccaggatggagtgcaggggcatgatcatagctcactgtagccttgaactactggactcaagctaacctcctgcctcagcctcctcagtaggtgggactaccggcacttgccactacacctggctgatcttttttttgagatggaggcttgttctgtcgcccagcctggagtgcagtggtgcaatcttggctcactgcaactgccacctcctaggttcaagcaattcttctgcctcagcctcccgagtagatgggattacaggcacgtgccaccacacctggctgacttttgtatttttagtagagacggggtttcaccatgttagccacactggtcttgaaatcctgacctcaagtgatctgcccacctcggcctcccaaagtgctgggattacaggcatgagccacggcgcctgaccacacctggctaatctttttaaaaagtttttgtacagacagggtctccctatattggtcaggcttgtctcgaactcctgggttccagcaatcctccagcctcagccttcccaagtgctggtattacatggatgagccactgcacctggctaattttactttaaaggaatctttctactattttatcattaagtatgacatttgtgttttcagaacatatattccctaccaagttacaggagttaattttaattcccaacttaatagtattttagtgtcatctatgggtgttaaattccatcaagtgatttatcagcatatactgagataatccttatgagttttatctggtagttaattaaaatattttctaatattaaatcttccaaacatactcttctgttttttgagacagggtctagttctgtcacccagggtggagtacagtggtacgatctcagctcactgcaacttccgcctcctagattcaagtgattctcccgtcccagcctcccaagtagctgggattataggtgtcagttaccatgccctgctatttttttgtatttttagtagagaggggtttcaccatgttggccaggctggtctcaaactcctgacctcaggtgatccaccatctcagcctcctgaagtgctgggattataggtgtgagccaccgtgcctggccccatatatctctttttaagtgggcatactgccattataaataatagtgattctgctggtaatgaacaaaggatgctggatccactaatagtctgttaaacctaatatcatgactttcttgttagctatacattggtttgctataattccatttagaatttttaaacctatgttcacaaatatggatttttaaacctatgttcacaaatatggatttttaaacctatgttcacaaatatggtttgcaagtcattttttctcctaaatttctatttgatggggaagttgtaaaatattggggttatttttccttggattttccttataataactattcctgaaaagtctctggaatgtctttcttttctggggctggggtagaaggactagatagatttacaaaccagtaactcaatttctgttttgtaaaattttcatttcattaaataataagtcctaatcaagtattattctttcccacagtatgtgagtgctgtcctcaatactgtcaacacttctggcttctaccaggcaaggctgcatgtagatttgcatctgaaaaaacaacaaactaaaatctaaccctaggtagtagtaaactgaatataaactttctcttatgaatttattctgtcttctttggtacatcaataataatatacacctttacagtatttcccagattgggggatacactttagcaagtatctgcgattatttgtttatgtaagatgtcccttcccttctgtgaatcatcattcttcaccccaagtatcttgagattggattctgtataagcagaatacaacagttaggcattcaggtatcattaaattcctccgcttcaaggatgaaaatttctttgggtatctaatagagtacaaagcagaaggtgtttcagaaatatttgcagtattgaatccgcatattcctccaagatagccctaatctaactggcagggtcccactcttcccagattaatgcccactcacataacaaacctgatgaggtagtgaagaaaactaactttgtgagtaagcaactggcagagtttttcaccactgtgactctatagctacatgtaactaagtagtatcactgacacataatcttaaattgaagttttaagatcattattctccatgttatacatgggtatcaaaagcattcccctcttgaccactccagaattctgtttaaaatttttcaatgacaacttatccatttccccaaagcctcagtgagcacatgatgccaacaattcatttcatgacttcatagcatgggccaagtttcttgcttaaaagacttccatcctgtcttgggaaacaaccatttccaaatatccacatatccttgcaagtttctgcctactcctctaccacccatttctgaagccatctgatttagtaagctgtatgcaaaagatacacaatggctaatgcaatcaaacaaggaatgtattaaaagcacacccaatagctcaaaataaaagacaagtgaacaaagttaagaaaatgacagtaacaaaagctgttctgggaacctctattgaaatagctacttattacatcaacatgctaccacagaacaaaagctcatgttgcttttctgaacttgaaaaacccattaacaatgtacagttctgagcctcagctgaccatagtgctcatgccaagtcctgagcagggcatcttgaatggtggttccctcatgactacatacaccgttagggaatgtttcgttaagaggaaatcaagatgttctaacctgtgaaggtagaatagattccaggctacacaaacacatgaagtgtgccttatattgattactaaagaggttgctgccaagactgcttccaaagggcagaagatagccctaaaaaatgtttgcagtgtggaaatgcatttttagtaagtcatattctagtaacaagttgcatttggtaagacacaaagaaacaatgttggtatgcagagtagaaatctctggaagatgatattgtcatatcagagatattgtcagtatcagagatactgaaatctctggaagatgatttttgtctcacatatggcattcgcaagtaaaatgccaaactgcaaaattcatattatgtagtacacataggaagatatctaaatatccctgtaggctctgggatgttatttcttattcttaacctccttactagattcacttgtacaatgaaataatctgtatcttattatttataattgagaattttctcaaaccttttcctgaaattttggaacacctggaataaaatttcttaaaatgattcctaaaagaaataattcttcaaaattaatattaagatataataacaggttggtttttttttttttttttttttttttttttagaatgaagcttctaaggtgaggttaacagtccagctgtggtttatttggtacattcataagatgttcactcctatatatattttttccctaggggtttctcatttctagatttacactttcccttatagcatggtccctccaaggtatatgcttccgatacataaaatgtttgtaattttgttaattctgccattcattagctcaataatttctctcattaaaattctgtaaactatgaatttcaaagaagtctattctatattcatctggttcatgaagtttcctctttgtgaatcttattttagtaaaatgactttacaacgtttaacatggttcctcacctgtatgaactttttaaaaaaaggtatgacttgctgctaaaaattttcagagtggttactaaattcagttttcctgtgtattgtctactatctttttgcatgtaaagaacagctttctgtggatgcctttccatatgctgtgcattcataaagtttctattcagtatgagttttctggaagatgacaagatgattccacttacagagtttctctttatatatgattgtttctatctcttgtgaatccacttttcagagtttcgtaaaattatcaatgtttgtcatctacatgagttctctgatgcataatgagctgtgacttccaacaaaaggctttcccacattcagtgcacttacaaggcttctctcctgtatgtgttctctgatgtgcactgagaattgatttttgagagaaggttttcccacattcattgcacccatagggtttctctcctgaatgagttctttgatgtacaatgagttgagaattcctaatgaaggcttttccacactcactgcattcatatggtttctctcttgtgtgcattctctggtgtacaagaaggcgtaatttcccactgaaggatttctcacattgactgcatttataagggttgacccctgcatgagttcgctcatgtacaatgagtagtgatttccaaatgaaggctttcccacattcattacattcatatggtttttcacctgaatgagttctcatgtgtataattaggtatgacttgctgctaaaagctttcccacattcactgcacccataaggcttttcccctgcatgagttcgctgatgtgaaatgagctggtctttcctattaaaggctttcccacattcactgcattcatagggattttctcctgtgtgaattctctgatgcacaatgagttgtgaattgaaactaaaggatttcccgcattccctgcactcatgtggtttctctcctgtatgagttctcatatgtataataaggtatgacttgctcctgaaggctttcccacactcactgcatccatatggttttactcctgtgtgacttctctgatgtacaatgagctgggacttcaaactaaaggtttttgcacattgactgcatccatagggttttactccagtgtgcactcctttatgtacaatgagctgtgatttgaacgtaaaggcttttccacattcattacaactatagggtttctctcctgtatgagttctctgatgtacaatcaggtttgactttgtattaaaggctttctgacactcactacattcaaatggtttctcccctgtatgagttctctggtgtataataagctgtgactttaaaccaaaagcctttccacagtcggtgcattcataaggcttctctcctgcatgagttctctggtgtgaaataagctggtatttccgactgaaggctttcccacattcatggcattcataggggttctctcctgtatgaatcctctgatgtataatgagctgtgatttaaaactgaaggctttcccacaattgttgcattcatggagtttttctcctgtatgagtccttgtatgtataataaggtatgacttgctcctgaaggctttgccacattcattgcatacataaggtttcattcctgtgtgacttctctgatgtacaatgagctgtgatttcaaactgaatcctttaccacactgaatacacccatagggctttactcctgtgtgaatcccctgatgtacaatgagctgtgacttgaatgtaaaggcttttccacaatcactacaaacataaggtttctcccctgtatgggttctctgatgtaccataaggtttgactttgtattaaaggctttctgacattcattgcattcatatggtttctctcctgtatgaattctttcatgtataatgagctgtgattttaaaccaaaagctttcccacattcattacacacatatggtttctgtcctgaatgagttttctggtgtgaaacaagctggtctttcctactgaagactttcccacattcacagcactcatagggattctcacctgtgtgaattctctgatgtataacaagctgtgaatggaaactgaatgttttcctgcattcactgcattcatgtagtttctctcctgtatgaattctctgatgtacaatgaggtatgatttactactgaagtctttcccacattcattacaaccatagggtttctcttcggcatgagtttgctgatgcactagaaggtatgacttgctgctgaaggctttctcacaacagctgcatccaaagggtttttcgcccatatacatttgttggcacataagttgcgatttcttattgacggtttttccagattcaatactttcacagtattttattccaataacagtttgctcatgtttagaatggaagaatgattttccatgtacctgaaacccattaggattatttctagcataatcactagtgaaatctatatatttcaaactctttccatgcgtgccacatttatgaggtttttgtcttgaaagatactttgtactaagaagacatagttttccaaatgtagtgcattcaaagctttttgccgtacttcccagcttgtctttattttcctgatgccaatccataagatcatcaattttccagactgtgtttggacaggtctgatttggaacttgggcctgcaccatacacagctcttctccttgttccaacttgaagatgatatcaggtttggtgtgttggtaccctagggacaccaggttgctatagttctccaacatcacactcctgtacaggcacttctgtgctgggtctagcagctgccactcctcccaggtaaaatccacaaacacatccatgaatgacaaaggtccccaggacttggtgatttttggctgctcttgggaaataaacagccactctaggactttctctattctgcgactcttctgcttctgcctgggtgttccagggagaggttgcagaccaggagtcccttggcccaagatggattcctgaccttggagctttctgatcctatcccatgaactgtttcgttcttggagaggtgggacccaaatagaagctgtccggaccctggtggccatccctacggtcagttttgtgtgcctcgctggaagtgacaggacgcgagggatgctccagatctgcagccagaagggttcgcaaccactccagactcggctggcccgttgaccacgacgggcgatgaacgctatctgaggaacaaggatctcgccatcggcgcggaacaatggcggccgctacgtat

SEQ ID NO: 18795 - RNA, 12678 nt, Homo sapiens
  source 1..12678: mol_type = other RNA
tgatatgtttgatattgggttgtctttttgttgttgggttgtaagagttctttatatgttctggatactagacccttatcaggtatattattttacagtgtcttttctcctatattcaccttttttttttttgagacggagtctcgctctgtcgcccaggctggagtgcagtggtgagatctgggctcactggttccaggttcacgccattctccttcctcagcctcccaagtagctgggactacaggcttccactaccagcctggctaattttttgtatttttttgtagagacagggtttcaccacattagccaggatggtttcgatctcctgacctcgtgatccacctgcctcagcctcccaaagtgctaggattacaggcgtgagccaccacacccggccttttttttttttttgagatggaattttgctttcttgctctgtcacctgggctggagtgcagtagcatgatctcggctcactgcaacctccacctcacagcttcaagcgatcctcctgcctcagcttcctgagttgctgggattacaggcacatgccaccacacccggcttttttttttctctttttttttatttttagtagagacgtggtttcaccaagttaaccaggctggtctcgcactcctgacctcaagtgatcctcccaccttggcctcccaaagtgctggaattacaggcgtgagccaccacacccagctccttttcactttcttgatagtgtccactgatgccgaaagttttcaattttggtgaagtccaatttacctattttttcttttgtttcccatgcttctggtgtcatatccaataaatcattgccaaatccagtgccaagaagtacatgaaaagattttcaacatcactagccattaggtaaaggaaaatcaaaaccacaatgagataccatttcatacatgttagagtggctattataaaaaatatggaggccaagtgcagtggttcaagcctgtaatcccagcactttgggaggccaaggtaagtggatcacttgaggacaggagtttgagactagcctggcctggccaacatggtgaaaccctgtctctactaaaaatacaaaaaatagccatacatggtggcacatgcctgtaatcccagctactcaggaggccgaggaaggagaatcacttaaacctaggaggcggaggttgcagtgagctgaaatggtgccactgcactccagcctgggtgacagagtgaaactccatttcaaaaaaaccaaaaaactatttgggtgtagtggcacctgtagttccagctacccaggaggctgaggtggaaggatcccttgagcccaggaggttggggctgcagtgagttatgatcatgcctatgaaatgagagagaaacaaactaattaatattggcaagtatgtggagaaattggaagccttgtgcactgctggtggaatgtaaaatgatagttgcacaataatggaaataatgtacttcatgccactgaagtgtacacttaaaaatagttaaaatggtaaatgttcttattatatatatgtgtatatatatgtgtatatgtgtatatatatgtgtatatatgtgtgtatgtgtgtgtgtatatatacatatatatatatatatatatatatatatatatatatatatatatatatatataaaatcacacatgaaagtctcccttggaactgatcctgaaataatttcatgtgtgatgaaagaacaccctgctctcctggagtgataagtggcctttttgttcatgctggcattatacatcccaggctcttccacacacacccagcataatttcaccaagcagagggagtacactctccaaaggcccatttgtgcctgtttctatcattatatcctcctatttaactcactccctgccctctacaaaccgtcatcaatcacagatatgtttgctacccctgtagtttctgcttttccataacatcatagaaataggatcatacagccttttcacactggtctctttcacttagcaatatgcctatcagattcatccatgtcctgcatggcctcagagcttgctcttgctgaacaggactccattgcatggatgtaccccagcctagttagtcattcacctattgaaggttatcctgattccttaaagtatttgtctgttatgaaaagagctgctgtacgtgagtacatgctgggttttgtttagatcaaactcctatgttttcaaagcagttatctaaatacctaggagtgtgattgttggctcatattgtgaagctttgtttagctttggggaaaagtcaaactatcttccaaagtggctatactattatgcattgcaccagcaatgaatgagagttcctgttgcaattgcaaatttacttatttttagattatagtcactttaatagatgtgcggtgctatctcgttgttttaatttgcttttccctcatgacaagtgtcactgagcattatttggtatgcttatttgccatctgtatatcttcttttttttttttttgagacggagtttcactcttgttgcccaggctggagtgcaatggcgcgatctcggctcacagcaacctccgcctcccgggttcaagccattctcctgcctccgcctccggagtagctaccacttggtggcagagtagcgccaccacgcctggctaattttgtatttttagtagagacagggtttctccatgttggtcaggctggtctcgaactccggacctcaggtgatctgcccgcctcggcctcccaaagtgctgggattacaggcgtgagccaccgtgcctggccaccatctgtatatctttggaaagtatgtatttggatctgtccccatttttaattgggttgtcttcttgttcaattttagggttttttttttatattttgcatacaaacactttttcagatttttttgaatgattttattcattacaaattccaattattgctatacattatttcaaatatataggaaatcacttgacttttgtctatggccatctactttgccttttattatctctatccattccaattaaggcatggaatgatggactctatttcagtttcgttttccaaaattatggcatggaaaatcgtaagattgaatttcaggggttcactgggactgcaagagggggcacatggccatcacaaaacaggaagcactgaccatccaacactgtgcctaggtagtaaggaaggggtgcaagcacacaccttgtctagcctgcttgcagtacctgcattctgctcacagacctctgggttgaatccacagaggaccaggccttccttctactcaggacctggggatcactagaggctgcatcacagtaaagactgagctgccttctcctcaggactgacctggggacccttggcaggggggaatccacagtgacaaacagaccttgcttctactcaggacccggagacccccgagggcacttcacagtgatgaccagaatttacctcatctcaggaccaacctgggggatgcatcacactgagaaccagagcttccttctccactggccaacctgaggaccactgtggggcacaaccacagtgaagactggagcttgtttctcttcaggactgacctagggaccctagtggggcaaatccacagtgaggttctgagcttccttctcctcaggaccaacctggggacccctgggaggtagatcacagtgatgaccagagtatcctcctcaggactgacccgtggtgggggatgcaaccacagtgaggactaaagcttccttttcctcacaacctggggaccccctagggggatacatcacagtgagatccagagcttccatatctgaagactcctgtagggtacacccacagtgacgaccagtgcactttccggaccaatctggggcgatgtcatctcacctttgggatacatggaggccacaggaggaaaagatgaggaaaagtgaggcctgcaccctgagtgctgaggagggagctttgctgtttcactttgccctgtaatatctgaacaagatttattttaggaaatcgtacctctattgaggtttccactagtcatctttatagcaagcccaactactttttatacatatgggtttgtttctggggagaaatcccagtacaaaaaaagggagaaacactgcgacaaaacactgcaacagtccaggtcaaagttggggatgaacagcacctgtgggatcaccctggatcccaagagggaagggcaaatgtgcaccctatgtgcttgcttttattaattttttttgaaggagtctcactctgctgcccgggctggagtgcaatggcacaatctcagctcactgcaacctccgcctctccagttcaagcaattctcctgagtagcttggattatagatgcatgccaccacagctggccaatttttgtatttttagtagagacggggtttcaccaggctggtctcgaactcctgacctcaagtcatccacctgcctcagcctcacaaaatgctgagattacaggcatgagccaccatgcccagcctttttattaatgttttaatggcctgtgtttctaacaagtagttgaaacaatgttgaaaattaaagagtagacatgttaaaacttgcaacttcatttaaatttaaatatatcatttataccaaaatcagaatttatttaagatttatggctgggtgcttggctcacacctgtaatcctagcactttgggaggccaaggcaggtggactgcttgagcccaggagtttgaaaccagactggaaaacatggtaaaaccccatctctacaagaaataaataactctacctggccctttagcaaagaattaagaaaaatcaatacagaccagtggctcacacctgtaatcccagcactttgggaggctgagggtggatcacgaggtcaggagttcaagaccagcctggccaacatggtgaaaccccatctctactaaaaacacaaaaattagctgggcgtggtggcgtgtgcctgtaattccagctactagggaggctgaggcaggagaattgcttgaacccaggaggcagaggttgcagtgagccaagaacacaccactgcactccagcctggcaatacagcgagactccatctcaaaaaaaaaaaaaaaaatgcaaatactatgccatataaggagcttgagcatccacagggagtatctgtggttgcgggggggtcctccatgaatactgacaactgcatacttgctactctactggcagttccaaacatttgtttgtggtttattttgggtttcctaattacacgatcacatctccaattcatggcagttgtttctgcacccatccctaattcctcacattccttgttttcacaccttggctagatgttactcatttcataaaagtgatgcgcattcttgtaattttgctttgttttttacagacagggtctcactttgttgcccaggatggagtgcaggggcatgatcatagctcactgtagccttgaactactggactcaagctaacctcctgcctcagcctcctcagtaggtgggactaccggcacttgccactacacctggctgatcttttttttgagatggaggcttgttctgtcgcccagcctggagtgcagtggtgcaatcttggctcactgcaactgccacctcctaggttcaagcaattcttctgcctcagcctcccgagtagatgggattacaggcacgtgccaccacacctggctgacttttgtatttttagtagagacggggtttcaccatgttagccacactggtcttgaaatcctgacctcaagtgatctgcccacctcggcctcccaaagtgctgggattacaggcatgagccacggcgcctgaccacacctggctaatctttttaaaaagtttttgtacagacagggtctccctatattggtcaggcttgtctcgaactcctgggttccagcaatcctccagcctcagccttcccaagtgctggtattacatggatgagccactgcacctggctaattttactttaaaggaatctttctactattttatcattaagtatgacatttgtgttttcagaacatatattccctaccaagttacaggagttaattttaattcccaacttaatagtattttagtgtcatctatgggtgttaaattccatcaagtgatttatcagcatatactgagataatccttatgagttttatctggtagttaattaaaatattttctaatattaaatcttccaaacatactcttctgttttttgagacagggtctagttctgtcacccagggtggagtacagtggtacgatctcagctcactgcaacttccgcctcctagattcaagtgattctcccgtcccagcctcccaagtagctgggattataggtgtcagttaccatgccctgctatttttttgtatttttagtagagaggggtttcaccatgttggccaggctggtctcaaactcctgacctcaggtgatccaccatctcagcctcctgaagtgctgggattataggtgtgagccaccgtgcctggccccatatatctctttttaagtgggcatactgccattataaataatagtgattctgctggtaatgaacaaaggatgctggatccactaatagtctgttaaacctaatatcatgactttcttgttagctatacattggtttgctataattccatttagaatttttaaacctatgttcacaaatatggatttttaaacctatgttcacaaatatggatttttaaacctatgttcacaaatatggtttgcaagtcattttttctcctaaatttctatttgatggggaagttgtaaaatattggggttatttttccttggattttccttataataactattcctgaaaagtctctggaatgtctttcttttctggggctggggtagaaggactagatagatttacaaaccagtaactcaatttctgttttgtaaaattttcatttcattaaataataagtcctaatcaagtattattctttcccacagtatgtgagtgctgtcctcaatactgtcaacacttctggcttctaccaggcaaggctgcatgtagatttgcatctgaaaaaacaacaaactaaaatctaaccctaggtagtagtaaactgaatataaactttctcttatgaatttattctgtcttctttggtacatcaataataatatacacctttacagtatttcccagattgggggatacactttagcaagtatctgcgattatttgtttatgtaagatgtcccttcccttctgtgaatcatcattcttcaccccaagtatcttgagattggattctgtataagcagaatacaacagttaggcattcaggtatcattaaattcctccgcttcaaggatgaaaatttctttgggtatctaatagagtacaaagcagaaggtgtttcagaaatatttgcagtattgaatccgcatattcctccaagatagccctaatctaactggcagggtcccactcttcccagattaatgcccactcacataacaaacctgatgaggtagtgaagaaaactaactttgtgagtaagcaactggcagagtttttcaccactgtgactctatagctacatgtaactaagtagtatcactgacacataatcttaaattgaagttttaagatcattattctccatgttatacatgggtatcaaaagcattcccctcttgaccactccagaattctgtttaaaatttttcaatgacaacttatccatttccccaaagcctcagtgagcacatgatgccaacaattcatttcatgacttcatagcatgggccaagtttcttgcttaaaagacttccatcctgtcttgggaaacaaccatttccaaatatccacatatccttgcaagtttctgcctactcctctaccacccatttctgaagccatctgatttagtaagctgtatgcaaaagatacacaatggctaatgcaatcaaacaaggaatgtattaaaagcacacccaatagctcaaaataaaagacaagtgaacaaagttaagaaaatgacagtaacaaaagctgttctgggaacctctattgaaatagctacttattacatcaacatgctaccacagaacaaaagctcatgttgcttttctgaacttgaaaaacccattaacaatgtacagttctgagcctcagctgaccatagtgctcatgccaagtcctgagcagggcatcttgaatggtggttccctcatgactacatacaccgttagggaatgtttcgttaagaggaaatcaagatgttctaacctgtgaaggtagaatagattccaggctacacaaacacatgaagtgtgccttatattgattactaaagaggttgctgccaagactgcttccaaagggcagaagatagccctaaaaaatgtttgcagtgtggaaatgcatttttagtaagtcatattctagtaacaagttgcatttggtaagacacaaagaaacaatgttggtatgcagagtagaaatctctggaagatgatattgtcatatcagagatattgtcagtatcagagatactgaaatctctggaagatgatttttgtctcacatatggcattcgcaagtaaaatgccaaactgcaaaattcatattatgtagtacacataggaagatatctaaatatccctgtaggctctgggatgttatttcttattcttaacctccttactagattcacttgtacaatgaaataatctgtatcttattatttataattgagaattttctcaaaccttttcctgaaattttggaacacctggaataaaatttcttaaaatgattcctaaaagaaataattcttcaaaattaatattaagatataataacaggttggtttttttttttttttttttttttttttttagaatgaagcttctaaggtgaggttaacagtccagctgtggtttatttggtacattcataagatgttcactcctatatatattttttccctaggggtttctcatttctagatttacactttcccttatagcatggtccctccaaggtatatgcttccgatacataaaatgtttgtaattttgttaattctgccattcattagctcaataatttctctcattaaaattctgtaaactatgaatttcaaagaagtctattctatattcatctggttcatgaagtttcctctttgtgaatcttattttagtaaaatgactttacaacgtttaacatggttcctcacctgtatgaactttttaaaaaaaggtatgacttgctgctaaaaattttcagagtggttactaaattcagttttcctgtgtattgtctactatctttttgcatgtaaagaacagctttctgtggatgcctttccatatgctgtgcattcataaagtttctattcagtatgagttttctggaagatgacaagatgattccacttacagagtttctctttatatatgattgtttctatctcttgtgaatccacttttcagagtttcgtaaaattatcaatgtttgtcatctacatgagttctctgatgcataatgagctgtgacttccaacaaaaggctttcccacattcagtgcacttacaaggcttctctcctgtatgtgttctctgatgtgcactgagaattgatttttgagagaaggttttcccacattcattgcacccatagggtttctctcctgaatgagttctttgatgtacaatgagttgagaattcctaatgaaggcttttccacactcactgcattcatatggtttctctcttgtgtgcattctctggtgtacaagaaggcgtaatttcccactgaaggatttctcacattgactgcatttataagggttgacccctgcatgagttcgctcatgtacaatgagtagtgatttccaaatgaaggctttcccacattcattacattcatatggtttttcacctgaatgagttctcatgtgtataattaggtatgacttgctgctaaaagctttcccacattcactgcacccataaggcttttcccctgcatgagttcgctgatgtgaaatgagctggtctttcctattaaaggctttcccacattcactgcattcatagggattttctcctgtgtgaattctctgatgcacaatgagttgtgaattgaaactaaaggatttcccgcattccctgcactcatgtggtttctctcctgtatgagttctcatatgtataataaggtatgacttgctcctgaaggctttcccacactcactgcatccatatggttttactcctgtgtgacttctctgatgtacaatgagctgggacttcaaactaaaggtttttgcacattgactgcatccatagggttttactccagtgtgcactcctttatgtacaatgagctgtgatttgaacgtaaaggcttttccacattcattacaactatagggtttctctcctgtatgagttctctgatgtacaatcaggtttgactttgtattaaaggctttctgacactcactacattcaaatggtttctcccctgtatgagttctctggtgtataataagctgtgactttaaaccaaaagcctttccacagtcggtgcattcataaggcttctctcctgcatgagttctctggtgtgaaataagctggtatttccgactgaaggctttcccacattcatggcattcataggggttctctcctgtatgaatcctctgatgtataatgagctgtgatttaaaactgaaggctttcccacaattgttgcattcatggagtttttctcctgtatgagtccttgtatgtataataaggtatgacttgctcctgaaggctttgccacattcattgcatacataaggtttcattcctgtgtgacttctctgatgtacaatgagctgtgatttcaaactgaatcctttaccacactgaatacacccatagggctttactcctgtgtgaatcccctgatgtacaatgagctgtgacttgaatgtaaaggcttttccacaatcactacaaacataaggtttctcccctgtatgggttctctgatgtaccataaggtttgactttgtattaaaggctttctgacattcattgcattcatatggtttctctcctgtatgaattctttcatgtataatgagctgtgattttaaaccaaaagctttcccacattcattacacacatatggtttctgtcctgaatgagttttctggtgtgaaacaagctggtctttcctactgaagactttcccacattcacagcactcatagggattctcacctgtgtgaattctctgatgtataacaagctgtgaatggaaactgaatgttttcctgcattcactgcattcatgtagtttctctcctgtatgaattctctgatgtacaatgaggtatgatttactactgaagtctttcccacattcattacaaccatagggtttctcttcggcatgagtttgctgatgcactagaaggtatgacttgctgctgaaggctttctcacaacagctgcatccaaagggtttttcgcccatatacatttgttggcacataagttgcgatttcttattgacggtttttccagattcaatactttcacagtattttattccaataacagtttgctcatgtttagaatggaagaatgattttccatgtacctgaaacccattaggattatttctagcataatcactagtgaaatctatatatttcaaactctttccatgcgtgccacatttatgaggtttttgtcttgaaagatactttgtactaagaagacatagttttccaaatgtagtgcattcaaagctttttgccgtacttcccagcttgtctttattttcctgatgccaatccataagatcatcaattttccagactgtgtttggacaggtctgatttggaacttgggcctgcaccatacacagctcttctccttgttccaacttgaagatgatatcaggtttggtgtgttggtaccctagggacaccaggttgctatagttctccaacatcacactcctgtacaggcacttctgtgctgggtctagcagctgccactcctcccaggtaaaatccacaaacacatccatgaatgacaaaggtccccaggacttggtgatttttggctgctcttgggaaataaacagccactctaggactttctctattctgcgactcttctgcttctgcctgggtgttccagggagaggttgcagaccaggagtcccttggcccaagatggattcctgaccttggagctttctgatcctatcccatgaactgtttcgttcttggagaggtgggacccaaatagaagctgtccggaccctggtggccatccctacggtcagttttgtgtgcctcgctggaagtgacaggacgcgagggatgctccggctcctccaaaccctgaaggggcagcagaatagagtccagggtactgcctccacctccagatctgcagccagaagggttcgcaaccactccagactcggctggcccgttgaccacgacgggcgatgaacgctatctgaggaacaaggatctcgccatcggcgcggaacaatggcggccgctacgtat

SEQ ID NO: 18796 - RNA, 12626 nt, Homo sapiens
  source 1..12626: mol_type = other RNA
tgatatgtttgatattgggttgtctttttgttgttgggttgtaagagttctttatatgttctggatactagacccttatcaggtatattattttacagtgtcttttctcctatattcaccttttttttttttgagacggagtctcgctctgtcgcccaggctggagtgcagtggtgagatctgggctcactggttccaggttcacgccattctccttcctcagcctcccaagtagctgggactacaggcttccactaccagcctggctaattttttgtatttttttgtagagacagggtttcaccacattagccaggatggtttcgatctcctgacctcgtgatccacctgcctcagcctcccaaagtgctaggattacaggcgtgagccaccacacccggccttttttttttttttgagatggaattttgctttcttgctctgtcacctgggctggagtgcagtagcatgatctcggctcactgcaacctccacctcacagcttcaagcgatcctcctgcctcagcttcctgagttgctgggattacaggcacatgccaccacacccggcttttttttttctctttttttttatttttagtagagacgtggtttcaccaagttaaccaggctggtctcgcactcctgacctcaagtgatcctcccaccttggcctcccaaagtgctggaattacaggcgtgagccaccacacccagctccttttcactttcttgatagtgtccactgatgccgaaagttttcaattttggtgaagtccaatttacctattttttcttttgtttcccatgcttctggtgtcatatccaataaatcattgccaaatccagtgccaagaagtacatgaaaagattttcaacatcactagccattaggtaaaggaaaatcaaaaccacaatgagataccatttcatacatgttagagtggctattataaaaaatatggaggccaagtgcagtggttcaagcctgtaatcccagcactttgggaggccaaggtaagtggatcacttgaggacaggagtttgagactagcctggcctggccaacatggtgaaaccctgtctctactaaaaatacaaaaaatagccatacatggtggcacatgcctgtaatcccagctactcaggaggccgaggaaggagaatcacttaaacctaggaggcggaggttgcagtgagctgaaatggtgccactgcactccagcctgggtgacagagtgaaactccatttcaaaaaaaccaaaaaactatttgggtgtagtggcacctgtagttccagctacccaggaggctgaggtggaaggatcccttgagcccaggaggttggggctgcagtgagttatgatcatgcctatgaaatgagagagaaacaaactaattaatattggcaagtatgtggagaaattggaagccttgtgcactgctggtggaatgtaaaatgatagttgcacaataatggaaataatgtacttcatgccactgaagtgtacacttaaaaatagttaaaatggtaaatgttcttattatatatatgtgtatatatatgtgtatatgtgtatatatatgtgtatatatgtgtgtatgtgtgtgtgtatatatacatatatatatatatatatatatatatatatatatatatatatatatatatataaaatcacacatgaaagtctcccttggaactgatcctgaaataatttcatgtgtgatgaaagaacaccctgctctcctggagtgataagtggcctttttgttcatgctggcattatacatcccaggctcttccacacacacccagcataatttcaccaagcagagggagtacactctccaaaggcccatttgtgcctgtttctatcattatatcctcctatttaactcactccctgccctctacaaaccgtcatcaatcacagatatgtttgctacccctgtagtttctgcttttccataacatcatagaaataggatcatacagccttttcacactggtctctttcacttagcaatatgcctatcagattcatccatgtcctgcatggcctcagagcttgctcttgctgaacaggactccattgcatggatgtaccccagcctagttagtcattcacctattgaaggttatcctgattccttaaagtatttgtctgttatgaaaagagctgctgtacgtgagtacatgctgggttttgtttagatcaaactcctatgttttcaaagcagttatctaaatacctaggagtgtgattgttggctcatattgtgaagctttgtttagctttggggaaaagtcaaactatcttccaaagtggctatactattatgcattgcaccagcaatgaatgagagttcctgttgcaattgcaaatttacttatttttagattatagtcactttaatagatgtgcggtgctatctcgttgttttaatttgcttttccctcatgacaagtgtcactgagcattatttggtatgcttatttgccatctgtatatcttcttttttttttttttgagacggagtttcactcttgttgcccaggctggagtgcaatggcgcgatctcggctcacagcaacctccgcctcccgggttcaagccattctcctgcctccgcctccggagtagctaccacttggtggcagagtagcgccaccacgcctggctaattttgtatttttagtagagacagggtttctccatgttggtcaggctggtctcgaactccggacctcaggtgatctgcccgcctcggcctcccaaagtgctgggattacaggcgtgagccaccgtgcctggccaccatctgtatatctttggaaagtatgtatttggatctgtccccatttttaattgggttgtcttcttgttcaattttagggttttttttttatattttgcatacaaacactttttcagatttttttgaatgattttattcattacaaattccaattattgctatacattatttcaaatatataggaaatcacttgacttttgtctatggccatctactttgccttttattatctctatccattccaattaaggcatggaatgatggactctatttcagtttcgttttccaaaattatggcatggaaaatcgtaagattgaatttcaggggttcactgggactgcaagagggggcacatggccatcacaaaacaggaagcactgaccatccaacactgtgcctaggtagtaaggaaggggtgcaagcacacaccttgtctagcctgcttgcagtacctgcattctgctcacagacctctgggttgaatccacagaggaccaggccttccttctactcaggacctggggatcactagaggctgcatcacagtaaagactgagctgccttctcctcaggactgacctggggacccttggcaggggggaatccacagtgacaaacagaccttgcttctactcaggacccggagacccccgagggcacttcacagtgatgaccagaatttacctcatctcaggaccaacctgggggatgcatcacactgagaaccagagcttccttctccactggccaacctgaggaccactgtggggcacaaccacagtgaagactggagcttgtttctcttcaggactgacctagggaccctagtggggcaaatccacagtgaggttctgagcttccttctcctcaggaccaacctggggacccctgggaggtagatcacagtgatgaccagagtatcctcctcaggactgacccgtggtgggggatgcaaccacagtgaggactaaagcttccttttcctcacaacctggggaccccctagggggatacatcacagtgagatccagagcttccatatctgaagactcctgtagggtacacccacagtgacgaccagtgcactttccggaccaatctggggcgatgtcatctcacctttgggatacatggaggccacaggaggaaaagatgaggaaaagtgaggcctgcaccctgagtgctgaggagggagctttgctgtttcactttgccctgtaatatctgaacaagatttattttaggaaatcgtacctctattgaggtttccactagtcatctttatagcaagcccaactactttttatacatatgggtttgtttctggggagaaatcccagtacaaaaaaagggagaaacactgcgacaaaacactgcaacagtccaggtcaaagttggggatgaacagcacctgtgggatcaccctggatcccaagagggaagggcaaatgtgcaccctatgtgcttgcttttattaattttttttgaaggagtctcactctgctgcccgggctggagtgcaatggcacaatctcagctcactgcaacctccgcctctccagttcaagcaattctcctgagtagcttggattatagatgcatgccaccacagctggccaatttttgtatttttagtagagacggggtttcaccaggctggtctcgaactcctgacctcaagtcatccacctgcctcagcctcacaaaatgctgagattacaggcatgagccaccatgcccagcctttttattaatgttttaatggcctgtgtttctaacaagtagttgaaacaatgttgaaaattaaagagtagacatgttaaaacttgcaacttcatttaaatttaaatatatcatttataccaaaatcagaatttatttaagatttatggctgggtgcttggctcacacctgtaatcctagcactttgggaggccaaggcaggtggactgcttgagcccaggagtttgaaaccagactggaaaacatggtaaaaccccatctctacaagaaataaataactctacctggccctttagcaaagaattaagaaaaatcaatacagaccagtggctcacacctgtaatcccagcactttgggaggctgagggtggatcacgaggtcaggagttcaagaccagcctggccaacatggtgaaaccccatctctactaaaaacacaaaaattagctgggcgtggtggcgtgtgcctgtaattccagctactagggaggctgaggcaggagaattgcttgaacccaggaggcagaggttgcagtgagccaagaacacaccactgcactccagcctggcaatacagcgagactccatctcaaaaaaaaaaaaaaaaatgcaaatactatgccatataaggagcttgagcatccacagggagtatctgtggttgcgggggggtcctccatgaatactgacaactgcatacttgctactctactggcagttccaaacatttgtttgtggtttattttgggtttcctaattacacgatcacatctccaattcatggcagttgtttctgcacccatccctaattcctcacattccttgttttcacaccttggctagatgttactcatttcataaaagtgatgcgcattcttgtaattttgctttgttttttacagacagggtctcactttgttgcccaggatggagtgcaggggcatgatcatagctcactgtagccttgaactactggactcaagctaacctcctgcctcagcctcctcagtaggtgggactaccggcacttgccactacacctggctgatcttttttttgagatggaggcttgttctgtcgcccagcctggagtgcagtggtgcaatcttggctcactgcaactgccacctcctaggttcaagcaattcttctgcctcagcctcccgagtagatgggattacaggcacgtgccaccacacctggctgacttttgtatttttagtagagacggggtttcaccatgttagccacactggtcttgaaatcctgacctcaagtgatctgcccacctcggcctcccaaagtgctgggattacaggcatgagccacggcgcctgaccacacctggctaatctttttaaaaagtttttgtacagacagggtctccctatattggtcaggcttgtctcgaactcctgggttccagcaatcctccagcctcagccttcccaagtgctggtattacatggatgagccactgcacctggctaattttactttaaaggaatctttctactattttatcattaagtatgacatttgtgttttcagaacatatattccctaccaagttacaggagttaattttaattcccaacttaatagtattttagtgtcatctatgggtgttaaattccatcaagtgatttatcagcatatactgagataatccttatgagttttatctggtagttaattaaaatattttctaatattaaatcttccaaacatactcttctgttttttgagacagggtctagttctgtcacccagggtggagtacagtggtacgatctcagctcactgcaacttccgcctcctagattcaagtgattctcccgtcccagcctcccaagtagctgggattataggtgtcagttaccatgccctgctatttttttgtatttttagtagagaggggtttcaccatgttggccaggctggtctcaaactcctgacctcaggtgatccaccatctcagcctcctgaagtgctgggattataggtgtgagccaccgtgcctggccccatatatctctttttaagtgggcatactgccattataaataatagtgattctgctggtaatgaacaaaggatgctggatccactaatagtctgttaaacctaatatcatgactttcttgttagctatacattggtttgctataattccatttagaatttttaaacctatgttcacaaatatggatttttaaacctatgttcacaaatatggatttttaaacctatgttcacaaatatggtttgcaagtcattttttctcctaaatttctatttgatggggaagttgtaaaatattggggttatttttccttggattttccttataataactattcctgaaaagtctctggaatgtctttcttttctggggctggggtagaaggactagatagatttacaaaccagtaactcaatttctgttttgtaaaattttcatttcattaaataataagtcctaatcaagtattattctttcccacagtatgtgagtgctgtcctcaatactgtcaacacttctggcttctaccaggcaaggctgcatgtagatttgcatctgaaaaaacaacaaactaaaatctaaccctaggtagtagtaaactgaatataaactttctcttatgaatttattctgtcttctttggtacatcaataataatatacacctttacagtatttcccagattgggggatacactttagcaagtatctgcgattatttgtttatgtaagatgtcccttcccttctgtgaatcatcattcttcaccccaagtatcttgagattggattctgtataagcagaatacaacagttaggcattcaggtatcattaaattcctccgcttcaaggatgaaaatttctttgggtatctaatagagtacaaagcagaaggtgtttcagaaatatttgcagtattgaatccgcatattcctccaagatagccctaatctaactggcagggtcccactcttcccagattaatgcccactcacataacaaacctgatgaggtagtgaagaaaactaactttgtgagtaagcaactggcagagtttttcaccactgtgactctatagctacatgtaactaagtagtatcactgacacataatcttaaattgaagttttaagatcattattctccatgttatacatgggtatcaaaagcattcccctcttgaccactccagaattctgtttaaaatttttcaatgacaacttatccatttccccaaagcctcagtgagcacatgatgccaacaattcatttcatgacttcatagcatgggccaagtttcttgcttaaaagacttccatcctgtcttgggaaacaaccatttccaaatatccacatatccttgcaagtttctgcctactcctctaccacccatttctgaagccatctgatttagtaagctgtatgcaaaagatacacaatggctaatgcaatcaaacaaggaatgtattaaaagcacacccaatagctcaaaataaaagacaagtgaacaaagttaagaaaatgacagtaacaaaagctgttctgggaacctctattgaaatagctacttattacatcaacatgctaccacagaacaaaagctcatgttgcttttctgaacttgaaaaacccattaacaatgtacagttctgagcctcagctgaccatagtgctcatgccaagtcctgagcagggcatcttgaatggtggttccctcatgactacatacaccgttagggaatgtttcgttaagaggaaatcaagatgttctaacctgtgaaggtagaatagattccaggctacacaaacacatgaagtgtgccttatattgattactaaagaggttgctgccaagactgcttccaaagggcagaagatagccctaaaaaatgtttgcagtgtggaaatgcatttttagtaagtcatattctagtaacaagttgcatttggtaagacacaaagaaacaatgttggtatgcagagtagaaatctctggaagatgatattgtcatatcagagatattgtcagtatcagagatactgaaatctctggaagatgatttttgtctcacatatggcattcgcaagtaaaatgccaaactgcaaaattcatattatgtagtacacataggaagatatctaaatatccctgtaggctctgggatgttatttcttattcttaacctccttactagattcacttgtacaatgaaataatctgtatcttattatttataattgagaattttctcaaaccttttcctgaaattttggaacacctggaataaaatttcttaaaatgattcctaaaagaaataattcttcaaaattaatattaagatataataacaggttggtttttttttttttttttttttttttttttagaatgaagcttctaaggtgaggttaacagtccagctgtggtttatttggtacattcataagatgttcactcctatatatattttttccctaggggtttctcatttctagatttacactttcccttatagcatggtccctccaaggtatatgcttccgatacataaaatgtttgtaattttgttaattctgccattcattagctcaataatttctctcattaaaattctgtaaactatgaatttcaaagaagtctattctatattcatctggttcatgaagtttcctctttgtgaatcttattttagtaaaatgactttacaacgtttaacatggttcctcacctgtatgaactttttaaaaaaaggtatgacttgctgctaaaaattttcagagtggttactaaattcagttttcctgtgtattgtctactatctttttgcatgtaaagaacagctttctgtggatgcctttccatatgctgtgcattcataaagtttctattcagtatgagttttctggaagatgacaagatgattccacttacagagtttctctttatatatgattgtttctatctcttgtgaatccacttttcagagtttcgtaaaattatcaatgtttgtcatctacatgagttctctgatgcataatgagctgtgacttccaacaaaaggctttcccacattcagtgcacttacaaggcttctctcctgtatgtgttctctgatgtgcactgagaattgatttttgagagaaggttttcccacattcattgcacccatagggtttctctcctgaatgagttctttgatgtacaatgagttgagaattcctaatgaaggcttttccacactcactgcattcatatggtttctctcttgtgtgcattctctggtgtacaagaaggcgtaatttcccactgaaggatttctcacattgactgcatttataagggttgacccctgcatgagttcgctcatgtacaatgagtagtgatttccaaatgaaggctttcccacattcattacattcatatggtttttcacctgaatgagttctcatgtgtataattaggtatgacttgctgctaaaagctttcccacattcactgcacccataaggcttttcccctgcatgagttcgctgatgtgaaatgagctggtctttcctattaaaggctttcccacattcactgcattcatagggattttctcctgtgtgaattctctgatgcacaatgagttgtgaattgaaactaaaggatttcccgcattccctgcactcatgtggtttctctcctgtatgagttctcatatgtataataaggtatgacttgctcctgaaggctttcccacactcactgcatccatatggttttactcctgtgtgacttctctgatgtacaatgagctgggacttcaaactaaaggtttttgcacattgactgcatccatagggttttactccagtgtgcactcctttatgtacaatgagctgtgatttgaacgtaaaggcttttccacattcattacaactatagggtttctctcctgtatgagttctctgatgtacaatcaggtttgactttgtattaaaggctttctgacactcactacattcaaatggtttctcccctgtatgagttctctggtgtataataagctgtgactttaaaccaaaagcctttccacagtcggtgcattcataaggcttctctcctgcatgagttctctggtgtgaaataagctggtatttccgactgaaggctttcccacattcatggcattcataggggttctctcctgtatgaatcctctgatgtataatgagctgtgatttaaaactgaaggctttcccacaattgttgcattcatggagtttttctcctgtatgagtccttgtatgtataataaggtatgacttgctcctgaaggctttgccacattcattgcatacataaggtttcattcctgtgtgacttctctgatgtacaatgagctgtgatttcaaactgaatcctttaccacactgaatacacccatagggctttactcctgtgtgaatcccctgatgtacaatgagctgtgacttgaatgtaaaggcttttccacaatcactacaaacataaggtttctcccctgtatgggttctctgatgtaccataaggtttgactttgtattaaaggctttctgacattcattgcattcatatggtttctctcctgtatgaattctttcatgtataatgagctgtgattttaaaccaaaagctttcccacattcattacacacatatggtttctgtcctgaatgagttttctggtgtgaaacaagctggtctttcctactgaagactttcccacattcacagcactcatagggattctcacctgtgtgaattctctgatgtataacaagctgtgaatggaaactgaatgttttcctgcattcactgcattcatgtagtttctctcctgtatgaattctctgatgtacaatgaggtatgatttactactgaagtctttcccacattcattacaaccatagggtttctcttcggcatgagtttgctgatgcactagaaggtatgacttgctgctgaaggctttctcacaacagctgcatccaaagggtttttcgcccatatacatttgttggcacataagttgcgatttcttattgacggtttttccagattcaatactttcacagtattttattccaataacagtttgctcatgtttagaatggaagaatgattttccatgtacctgaaacccattaggattatttctagcataatcactagtgaaatctatatatttcaaactctttccatgcgtgccacatttatgaggtttttgtcttgaaagatactttgtactaagaagacatagttttccaaatgtagtgcattcaaagctttttgccgtacttcccagcttgtctttattttcctgatgccaatccataagatcatcaattttccagactgtgtttggacaggtctgatttggaacttgggcctgcaccatacacagctcttctccttgttccaacttgaagatgatatcaggtttggtgtgttggtaccctagggacaccaggttgctatagttctccaacatcacactcctgtacaggcacttctgtgctgggtctagcagctgccactcctcccaggtaaaatccacaaacacatccatgaatgacaaaggtccccaggacttggtgatttttggctgctcttgggaaataaacagccactctaggactttctctattctgcgactcttctgcttctgcctgggtgttccagggagaggttgcagaccaggagtcccttggcccaagatggattcctgaccttggagctttctgatcctatcccatgaactgtttcgttcttggagaggtgggacctgtggaccaaatagaagctgtccggaccctggtggccatccctacggtcagttttgtgtgcctcgctggaagtgacaggacgcgagggatgctccagatctgcagccagaagggttcgcaaccactccagactcggctggcccgttgaccacgacgggcgatgaacgctatctgaggaacaaggatctcgccatcggcgcggaacaatggcggccgctacgtat

SEQ ID NO: 18797 - RNA, 13145 nt, Homo sapiens
  source 1..13145: mol_type = other RNA
tgatggataaaagactacatattgggtacagtgtactctgctagggtcatgggtacatcaaaatctcagaaatcaccactaaagaacttatccatgtaagcaaacaccacctgttccccaaaaactattgaaataaaaaataataacaataaatatctttaaaaatatgactctatttaaatgttgagataaaatgaggctctattttccacgaagaaattaataatgctaaaattaagaattccagtttctccaataaacaattatatatttaacaaaaagtagtttattaatcacctttgttattgctgatatttatcccattgatttagaatcactactgccttcctgagagctaaacatctctttaatcaaataacatttttattttttgcttattatttgaacatgtgccttaaaagcactgcctattttgtttctaataagatatttatttttacctattttttacattgcagatttgttccactgttgttgttgtttttgtttcaggtatagaatgccacatactacataaaatgattctttttgcttatgaataatgtcaccaatttttaaaataacttgcagaaaacaaaactatgactaggcgttttcagtaaaaatgctaacattttggcaactttgtgaaattgtttattcctcctgatggtgtatacaacagagaaatgtggagaaaatgttctactaagaactcaatgataatttgctctacctatcacattttttaaattccatgtggttgtctccattaacggatggttaaacagctccaatttgaagacaaaatctttgattttttaggaaacaaatttttggagtatcagataatcattagttttcttatgacttgcaaaaaatttaccttggttatagtggtagctagggtcagacagattaattatattaaggctagacagtactatttttgaaggtagtttctcttcccttttaatagtaatgaattatttaaacaggaatcatgtaactaacacttagcactgttctaagaactttccgtatattacctcaattaattatcatgtaaatccagcaagttaataacttttaaaactcctattttacagataaacaatttgtagcacaaagagataaacagcttgcccaaagtcacacagctaggaagggggatcccagaattaaaactcaagcattctgcacttaaaattactacacaatactggcccactagcttaccatgttccatggcagaatccaatcattttacccacggccattctttaataatggcttcgaacttcttactccatgacctttgctgcttattttctcatgcacaccacagaccacactggactcattccttccacaagaactctgccccttgaatagagaagagcttttaaaatcgtaagtcaggactcacatcttctctataatattctccctaagtgtagtaaaccattgaaatgttcaatattatatgcctattctaattacttggagtagttgtcaataatacagtattgagaaatatcttgagaaaaaaaactagccttactagataagtgcttgatcattagcaacttttgttctgaccacagaacaactcatagcaagctgtaagtttgttccccctgctactgaaaccaatgccaaagtatgaaatatgttaccttgctcctaaaagcaatgagacataaaatagttggcttaataataacattaaaaaattctatttaaaagcaagctatacttcattatccccatcttctgatttaatatattagataggcatttatctataaacttacttgatcaaatatttgagtgaccatgatacccaaggcactgtgctggtactgcagagaatacagggccgaggaaatgatcttgtactcaagtatagaaagcagaacactttttttttttgtgaagatatgatggttacagtagtatgactgttagatgcatgaactcagataggacagacatacaatcaaccacataaggcagaaactgataaatactaaaagaaaaaaaaacaaatattaggcagaaatgtggaatattattgaatcatatattcaaatataataattaaaataaatctaacataagaataagaatgtgagaggatgcaatgtgggaaactacttaaagcttgaggagataacatgtatcaataatgtgaacaagagcatggagggaagcccaagccaaagaaagcaataagcactgcatgggcaaggagaatcaggaagggaagctcccccagcctgcagcagagtggtgcctaactagtgatttgtgaagatggctaaaaggaggaggtgtgctgtgagagggcagcgcaggcacaggcacttgcaccatcaatgacatcttgaccctacagagccaaatggagatgggcgtccagctcccaggaggtggatttgtggatctaagcctcatgttacttctcagctgaattgaaagaaacagctacaaatccccaaagtacaaagagatgctaagcaagaacaggtgttcttgtggccagagcatcaaaagcaacacgtacctgtcatgtcccacttgaggagaaactagttctacttgtatgcaagtatgtgagtgataaatacataaatggttatgaatgctaacaaagtgctgtttattggaatttggagtctcagaaattggctcttcactcaaagatttcaaaataatgcactcctgcttttagttagcattaactatattttttatcagttggaaaatagctacctatgtaatagagaacatcgaactgaagaaaaccagagaagacttcataaaggaaagttctctcccattttctccctcctgctaaactgctccaacccctttctcactttcttccaaaatacaaatgtcctcctaaacagccctcttttctgagttgcagatcaaatgtctggaaatcctccatctgcaggtgacaatgttgaaagatctagcaaggccttctcctcctgcaacattccatatatgaactaatgatatcaccacttctctgctgccatttctaaaccacaaggcttgcccagggcctctcaaaacccactgtccatgactgtatctccacttattttcccttagctaaaaatgtgttctcccctgaactgctttccctgtgccccttgtatcaaggttgctcattcttttcatcctcatatatttaagggtaaggagttcatatcagtgtcttcttcattccccatagtaccttctcaatcattcccaccccaatgtgtttgtaaaaatctatacctctctgaatctggtcccatttttctgtacaacttattgtggacatctgtgagttaccaacacagcattcattctatcatgtgcccttgttaactatacttcaatttttttcaacagtgacccatccccctacttatgccctaaagtcaactttttgataaactgactttagttctacctctagaattagtgtatgcatttacctggccacattgatggccttaggcataatcttatcagagtgaagctcaaaacttttgttcagtggttgcaggaaatggacactttttcttccacgagaggcaaactaggaagaatggattcaccattgctgctgatacctgtcttgcaaccaggaggaaaatcagcctaaagaaaaaactaacatataaaggaaagaagaaccaaagaaacaggaaaaaagaaaatgtagaaccaagacctgattgaatagttcctgaaacaactttacttgtggacttttctgtttgtctttaagtcacttgagatgggttttctgtactttcattgactttgtcatcactagaaactgttccttttcaaattcctactttaaaaatcctatcctcagacatcagcctcctgtcctttcagtttgttcacttacacatactacagtactaattagaatgtcatatctgttgaccatttttactatccacctactccttcctattttcatatataagttttgttcaccagtgggccaacccatgtagctcagtgtcttacatttagtaggcaattaataaattgtgttgattcattggttaattgattgttctctttgcctttctctctcaccccttcccaagtatgcttcacctagtgattattcttttaaattttttccataattatttttctgtaacacaatatatccttattactgtcccactggaaatcttcaataacactcattttgtccatagctggacctcagatgtggtccacactatgttcctgatgttgttgctttctaaaggttatcatcttccaattgagattgaggatggacaaacccttcctgaaccaaattcagtgctggaagccaccttaaaatgtcaacttcaaatatggtctaaaataatgtacttttaataaataaatataactctccatcatcacaaacctcagaaaagccatgcaatgatctctcctgcagtatctaattttgtaagaattccattctagacattatgctttaatggaacactggcaaaataaaagttatccaaagagtaaccaggatggtgaaaagcccagaaaccatgtgtcaaggggaaaacagggtttctttgcagagagagggtgtggggaccataacatttatgttctgatatttgaaggactgtcaagtggaagaacaaaagttgcaattctcttctgctccagacatcagaaaaagattaaatttaatcttatatggagttatatcttagctcaatatgaaatgtaacattaaaataatgtttctatccaggtatccagctataaaaggggcttacataaaagcagagttttataaagtatcaatcaagttagtctagtttgtgctgtagcaacaaagaacccccaaatctcaatggtatatcaaaaaaagtttgtttcttatttatactactttatttgtccagcacaggtcacaaaagatcctacgcattgtagccttcaaagactcaagatgacagaagatccaccatcctatgacactgccatctaaacacaagtctccagcggccactgtggcaaggaaacagagcttgaatcataaatcagctcttaaatgcttctgcctggaagtgattcacatcacttcacttaaatttcattggccaaagcagtccatggccatgtataatttcaaggagatgagacagctgtaaaaggaaggatgtcagaagcttcagttagcacttggaacatctaccataactttcagtaggatttaagcagaattcaaattctcattaggaatatcatagaaaaagttagattgctaagcctctttaaactctaggattctataattccaaacttatgtcagatagttcctttaatatcagggattttgcttcctagggtaaaatgaataactctggagcactgaaacttcccatatacaaaggactatgctcaatatttgaatttactgagctgagcttacaaagacttggcttggaagagctaaatattggcaggtcaacagccctaactctgtaagcttgttatggtccatttttttcaaacattgcttcaaatatttacatttgacttttacataaaagttgctgattttcagtagaggctgagatgaacgacagttgataactgttcctcatgttctatagaatttatgtgtaaggtttccagctatttttctatcttccttggtaagactgtagtgtagctaaacaggtggacttaaatgtcagctgtattctagtggcttaataatgcctttgaatacgtaatagccaatgcttacaggttatgttattttatattacagtctcctgtttaattttactgcagatacgtcttaaattgagagcaattactcccttcatttttgccattttaaacctgctgtgtactcattttttttaaattatgggccaaaaaaggacagctatacattttcagtgtcatggatctagagttatagctctagaggggccacagagatcacctagtttgcccctttgttttacatacaaaaaatttaagaacagttaacatttgttgagagtgtaccatgttctgggcactggcctactgttttctcatgtattaactcaactgatcttctcaatagcccaagaaaataaatactgtcatcatctccatttcacagatgaataaacttacctaagattgggaaacatttcccccttattagacaggtcaatattttaaaaaaaaaaatggcatagcctggtgctggggagaacacgaacaggcacatggcctcatttactgttcagcattttgtgacatttagctcaaactttttgatattgaatcttcctccatttctccacagttcttacatatcaatttggacaaaggtgacaagataatagcaaattccaagaaaaactattacatagttcaaataatcacacaattacatattagacagaaagtaaaggctagagaaagtctgcagcactacctaatctgagaaaatgattgggaaggaatgttaaaattattaaccattgaggcttgggccctaggctcccttactgggaagtttctggaatagtttctagagttatgtctgaaatagttttccaattctgattgaaacctttaagctaataatgcttacctatgaatgaagagatttgggtgacttttacatttttctttgtacttttcaatattgtttaattttccattgcagtgacaatacattttataaaatcatcgagaagatttaaacaaatgcaatgagtttattgaatgagctgaactcaggaagatagcaaaaagcaactttgttctttctcaccctgtacctgcatacctgttctttgggtttcatttaacaagctattctacaacctaagagataggcactaccctcccactcctgaggtctaccacttttagaactgtctactattgtcaacactacctgcgacccagtcttcggcatcccctcctcaaactcatccccctaaagttccagtctctgtcctgctcagacacctgtgtcagggctctctccagtgattctgaattgagtgcccttgggcacccctggtaagagcctctgtctactcaaccacacccagagctaccattcgctgtatgaagctggaaaagttcacaccccttagctctggtgctgaagtggacacgggtagagcacaggaaaatgtgctccctacatcccaaatgaaagccctgaactaatagaaacaaatgatgaggaggctctgtatcactgaagtatggacacattgtgggttaaaggctttggcagactgaactggagacataaccttcattcatcacacaatttctatagaaaaatgtgtcgagttcaaaacaactgacctacaaatgatccttaggaacataatttgtctggaaactgggggctgcttttataaccatctccagcctgtcagatccaatagattagagtcaagacagcacctttgatttacagtcttggccctgttgctgaagcacttcctaattcacactctctattcttaaaatgagaggcataatatgtctgctccaactacaaggttgttgagataataagcatggctatttctgagaaaatatcttacaaaattgacaatataagtgtttactattatttcatgtggtgcattacagaattcacagtacaggtaattggttatagggaagtcgtttctgagattaataagactgccgcaaaagtatcacaatatgctcctgttttttccccattcctgatttctttccttagcaaaaaatgttcctttgtctttcttaacctatgcatttttaggttattggcttttagaatattggcattactgaaaccctgtctaactttaggagcgctaattgagtatataataacacacatgtaaatcaacaaattttagaaagccttagaatctgcaaaaagcatgaaacataatttatcctatgctaagtacagtaactaggtaatgccagtgttaaaaaaaaaagtataaaacttgaaaataaggataaaagggtagagcaagcccttttgatgtctactggtatattatttcaatagtccacttcatgacaatttatctgattactcatgtttgactttgctatttcctatttgattagagactagacactatggaattatatgttaaattgtagatttttgttaagtaaaaaagataaccttaaagatggctgttctgttgtcccgtgggccactaaccaatgttgtatccaacccagctatcctattctaatatccttttaatgtctttcctgctgtactatatatatcattgttccttaaatgctcttggaaccagtttcatcctcatattggtatgtatgtatatgtatacatatatacacatatatgtatatatgtatacattatctgtaaacataataaagtgctttgaagaaattttaaaaataggaaagtgggtggtgccaaggaagctgagggaagaaaatgtttgagaagggaatgctcagaagaggctgcactgccataagttgaagggacttagcagtaaggaataggtcagtaaccttggagagagcagcattcatggggtggtgaaggcagaaaccgcatcattaagagcaaggggaagagggccagaacgtacacaccactttagggaagttggaatgtggggagagcagtgcaatgagatggtgccagatagataagagatccaaggagaggtatatattttgtgtgttttctgggttttttgatgttgtttgttttaatgggtgagaccagagtatatttaaatgcagatgggaagaacagtttgaagatcaagtaagagggatggaggtgggggtgaataattaaaagaaaaaagattcctgaggaggcaagaggggatagaatcccaagaacagatatttcagggtgggggcggggctggcaacagacagcatgttggctggctgaagttacggtgggaggtggtgggagttgtaagtctgaggagcttgtgaaatgtttcagatggaagctgtgggaaatagaagaaagctaaaaaacacacatgaattgcaaaatagcattgaggaccccagtacaagttgaatgcaatgacatcatagtggcaccaatatgattatatgaggtttttttttctccagccatgctcaagacttcagcttagccaaggaaatagcaggcacggtaggtattttctggctggttatgagtggaatataatgagagaaggtaaataggacacttatagggaggtaactgaagcaatggactaagcacttgtccaaacatttttgttctcatgctctcaaaagattttggaaaactatttctcacatattttgaaatcaaaatctaaaaatttttaacacataaagtgaaatagtttcaaaggatgtatttatggcttatattatatatgtacattaaatatatttttatccaagtcttggagttgtagatttagctcattctatttatagaacacgtctttcagataatcaggccacattgtgaaactaatcagccaaatcagggttacttttcatcagaaccagtacaattttattttaaaattcatacagtcatgcatctgtggaatacttctgtattctaagataggttaattgatttttaaatggatggttgattgttgggtagatagctggtggatagatgaataaaacaagacatggatggatagacaaattcttatcttgagtttgtctcctggataaaacaagatcccctcaaatatttctctctgaagtttttttttattttactttcaagagactttccctcaagaaagtggtattctagatttgtccctctttttgatgccccaagtgtttttacaccctggagcaatgcatcaaaatacaacttaggatgggggaagtacacttttcttttgtaaagtggagaagggcaatgtgaaaggtgaaaaaggaaagactaattggtagacatcagagtttgtatgcaggtcagcttgaagaatgaatatgaggaagttgagatttagaaatttctacactacagctttctaagcttttttgattatcccacaggtacctaaaacttaacatgcctaaaattgaacttacatatctacctcatcctagtcctccttcctcagtgagtggcaccatttctattcattaagacaagacagaaacctggcagtcaccctgaacttcttgttctctcatgcccttcatatccaactaaacaccaagatctggacattttttctcataatgatctcctgagtcagcccacatccctctatccccatggctatctctctgctgcagggtatggttgcctctcactcagctgccaaaatctgcctgtctctagtcttgagtcctctccacctgctctccatactacaaccagagaaagtattctaaaacatgtctgactaaatagctccatttttaaaaagttatcaatgacttcctataaccctaggccttattattcacttactagattactatttcaatcaagctctaaggacaaatcctaaactcattggcatggctttcaaggcccttctgaacttggcctctgctcatcatggcagcttccgctctccccactccatactctgcttatgaagtgttttcatcccaagtctcaccaggctctcctgcctcaaacactctttctgcctccttcttctagctccctcctatttagcattaaggtttcagctgagatgtaatttcctctagaaagcttttcctaatccctcaagtttgggtttgatccttatcttacatacttctgtgacgcattgtttgtagtccattatagcatttactctacattgagttttaactgtttacatgtctgaatacccaagagcagagggacatatgtgtgtgtctattcacttttgtattgtcagtgtctagggtactagccactgcctggtgcagagtaggtatccaataaacacgtacttaccgaataaatacgtgaagctaccaaaattttgcccccaaaataaatcacattccttctatgagtggcttataaacctgtttagtgaccaaatataaagttttcatcaagttcatatgaaattgttggcaaaaaataatccataagcttgatggggaaaaaattccatgccccatctctctaacaatgatatcaaaaactacttccttatacatagcaaaataacttagctgagaactgagtcaaaaggaactgaaattttcattattttattaattcattcaatgatcaatggtcacttagctctgccttcatgaagcagtgttgctctagtctagtctaatgcttgccccatgaagcccactgaaccctggagaaaagctggcccatctcttcagctttccaaattttattatatagaactaggagcagctgcttttatccaagtaggaataatttttaaatagcatttttccttgtatgtcagaaaacccaagctgaaaatattacatttcttaaaacttctatgctcctgatctttttcttcttttctgttgtgccagaggcatgaactttatgcccccagcaccagttaagaagatgatttattaaacagacttaaatgaaagatggcttggtgtggatacacttagattcacagaccgtgccttggggcagttttagtgccaactttctaactaattcagaaatgaaaaacttctcattatttcaggataaatgtctaaacctaccagctcttgtctgaatgacataaaagtatcagcactaaaaatggagattttgttgttcacatgtcatctagactctcaaccctacaatgtttaacatatgagccagttacaaattaccaactaatggtatcttttgggcacttccaggtaaagcctcccagtgtccattgtatcaaactctttccctttcatacagggttacctgtacagtagtatcactcagaagttatgctggaggaattgctttcaattttttcattaggttcataaaatctactcagaaaatagatttaaaacacaaatgttaaaatccatgcaaaaacacaaatattttgatttgatttatgcaaagccctaagcctgtgctgtgcacagagaagagagcaatggcatgactacttgtctgtttactctcagaatgtgcatatatgcatttcatttccttgatttgaccctaattcaaggggccagtctgaagagtcagcaatgttaatttactagatctcaaaagtaagtattcatattactgcaaaaagcaagatgtcattttctcatcatttctgtgaatagaaaagctattttccaacaatagggatcccttataatagggaaatacttaactggtactgaactcagaaactgcagtgttctgcttggcttcattgattttatcaaaggacctctttatcctgagcaggtaaagctcaatgaattgaaatagtccagaaatacatgaatagctgtcctctgacagaaagtaagtttaaattgtaagaaaattactttatttccaaggattcccgagattcttgttcctgattatggtccaaaattccacacagatttgttcttgattcatttcagagtagtcagaaaaggtactgttctccttacatagagaaagaacatcctgtggtttcatctcagaactgtagctctcatatttgcaacagaaaaaagctggaccaacagcacactaatggctttttgtgaacccatcagaaagctaaagtcgaaggataatagtcttcctgaaatctagagagatgtggggtacctatgtaaaaattagagggctgtggtggacacaggaatcataaaatcagccagtccttttgctgaaatacatttctagtagtgccatgggtgatttgaaaatagtcttgttccttttcttcattcccttgcacactctgtctcctcttctccatggctctcttgatgcagggaagtggcaaagttctagaagatcatcaagggctggaaatattgctgtggtcattccagagaaatgcaatagatgtgactgggcgcagcggccaccgtaaggcgtaaggggtgccaagtgccggttccagtcccgcccagcc

SEQ ID NO: 18798 - RNA, 13239 nt, Homo sapiens
  source 1..13239: mol_type = other RNA
tgatggataaaagactacatattgggtacagtgtactctgctagggtcatgggtacatcaaaatctcagaaatcaccactaaagaacttatccatgtaagcaaacaccacctgttccccaaaaactattgaaataaaaaataataacaataaatatctttaaaaatatgactctatttaaatgttgagataaaatgaggctctattttccacgaagaaattaataatgctaaaattaagaattccagtttctccaataaacaattatatatttaacaaaaagtagtttattaatcacctttgttattgctgatatttatcccattgatttagaatcactactgccttcctgagagctaaacatctctttaatcaaataacatttttattttttgcttattatttgaacatgtgccttaaaagcactgcctattttgtttctaataagatatttatttttacctattttttacattgcagatttgttccactgttgttgttgtttttgtttcaggtatagaatgccacatactacataaaatgattctttttgcttatgaataatgtcaccaatttttaaaataacttgcagaaaacaaaactatgactaggcgttttcagtaaaaatgctaacattttggcaactttgtgaaattgtttattcctcctgatggtgtatacaacagagaaatgtggagaaaatgttctactaagaactcaatgataatttgctctacctatcacattttttaaattccatgtggttgtctccattaacggatggttaaacagctccaatttgaagacaaaatctttgattttttaggaaacaaatttttggagtatcagataatcattagttttcttatgacttgcaaaaaatttaccttggttatagtggtagctagggtcagacagattaattatattaaggctagacagtactatttttgaaggtagtttctcttcccttttaatagtaatgaattatttaaacaggaatcatgtaactaacacttagcactgttctaagaactttccgtatattacctcaattaattatcatgtaaatccagcaagttaataacttttaaaactcctattttacagataaacaatttgtagcacaaagagataaacagcttgcccaaagtcacacagctaggaagggggatcccagaattaaaactcaagcattctgcacttaaaattactacacaatactggcccactagcttaccatgttccatggcagaatccaatcattttacccacggccattctttaataatggcttcgaacttcttactccatgacctttgctgcttattttctcatgcacaccacagaccacactggactcattccttccacaagaactctgccccttgaatagagaagagcttttaaaatcgtaagtcaggactcacatcttctctataatattctccctaagtgtagtaaaccattgaaatgttcaatattatatgcctattctaattacttggagtagttgtcaataatacagtattgagaaatatcttgagaaaaaaaactagccttactagataagtgcttgatcattagcaacttttgttctgaccacagaacaactcatagcaagctgtaagtttgttccccctgctactgaaaccaatgccaaagtatgaaatatgttaccttgctcctaaaagcaatgagacataaaatagttggcttaataataacattaaaaaattctatttaaaagcaagctatacttcattatccccatcttctgatttaatatattagataggcatttatctataaacttacttgatcaaatatttgagtgaccatgatacccaaggcactgtgctggtactgcagagaatacagggccgaggaaatgatcttgtactcaagtatagaaagcagaacactttttttttttgtgaagatatgatggttacagtagtatgactgttagatgcatgaactcagataggacagacatacaatcaaccacataaggcagaaactgataaatactaaaagaaaaaaaaacaaatattaggcagaaatgtggaatattattgaatcatatattcaaatataataattaaaataaatctaacataagaataagaatgtgagaggatgcaatgtgggaaactacttaaagcttgaggagataacatgtatcaataatgtgaacaagagcatggagggaagcccaagccaaagaaagcaataagcactgcatgggcaaggagaatcaggaagggaagctcccccagcctgcagcagagtggtgcctaactagtgatttgtgaagatggctaaaaggaggaggtgtgctgtgagagggcagcgcaggcacaggcacttgcaccatcaatgacatcttgaccctacagagccaaatggagatgggcgtccagctcccaggaggtggatttgtggatctaagcctcatgttacttctcagctgaattgaaagaaacagctacaaatccccaaagtacaaagagatgctaagcaagaacaggtgttcttgtggccagagcatcaaaagcaacacgtacctgtcatgtcccacttgaggagaaactagttctacttgtatgcaagtatgtgagtgataaatacataaatggttatgaatgctaacaaagtgctgtttattggaatttggagtctcagaaattggctcttcactcaaagatttcaaaataatgcactcctgcttttagttagcattaactatattttttatcagttggaaaatagctacctatgtaatagagaacatcgaactgaagaaaaccagagaagacttcataaaggaaagttctctcccattttctccctcctgctaaactgctccaacccctttctcactttcttccaaaatacaaatgtcctcctaaacagccctcttttctgagttgcagatcaaatgtctggaaatcctccatctgcaggtgacaatgttgaaagatctagcaaggccttctcctcctgcaacattccatatatgaactaatgatatcaccacttctctgctgccatttctaaaccacaaggcttgcccagggcctctcaaaacccactgtccatgactgtatctccacttattttcccttagctaaaaatgtgttctcccctgaactgctttccctgtgccccttgtatcaaggttgctcattcttttcatcctcatatatttaagggtaaggagttcatatcagtgtcttcttcattccccatagtaccttctcaatcattcccaccccaatgtgtttgtaaaaatctatacctctctgaatctggtcccatttttctgtacaacttattgtggacatctgtgagttaccaacacagcattcattctatcatgtgcccttgttaactatacttcaatttttttcaacagtgacccatccccctacttatgccctaaagtcaactttttgataaactgactttagttctacctctagaattagtgtatgcatttacctggccacattgatggccttaggcataatcttatcagagtgaagctcaaaacttttgttcagtggttgcaggaaatggacactttttcttccacgagaggcaaactaggaagaatggattcaccattgctgctgatacctgtcttgcaaccaggaggaaaatcagcctaaagaaaaaactaacatataaaggaaagaagaaccaaagaaacaggaaaaaagaaaatgtagaaccaagacctgattgaatagttcctgaaacaactttacttgtggacttttctgtttgtctttaagtcacttgagatgggttttctgtactttcattgactttgtcatcactagaaactgttccttttcaaattcctactttaaaaatcctatcctcagacatcagcctcctgtcctttcagtttgttcacttacacatactacagtactaattagaatgtcatatctgttgaccatttttactatccacctactccttcctattttcatatataagttttgttcaccagtgggccaacccatgtagctcagtgtcttacatttagtaggcaattaataaattgtgttgattcattggttaattgattgttctctttgcctttctctctcaccccttcccaagtatgcttcacctagtgattattcttttaaattttttccataattatttttctgtaacacaatatatccttattactgtcccactggaaatcttcaataacactcattttgtccatagctggacctcagatgtggtccacactatgttcctgatgttgttgctttctaaaggttatcatcttccaattgagattgaggatggacaaacccttcctgaaccaaattcagtgctggaagccaccttaaaatgtcaacttcaaatatggtctaaaataatgtacttttaataaataaatataactctccatcatcacaaacctcagaaaagccatgcaatgatctctcctgcagtatctaattttgtaagaattccattctagacattatgctttaatggaacactggcaaaataaaagttatccaaagagtaaccaggatggtgaaaagcccagaaaccatgtgtcaaggggaaaacagggtttctttgcagagagagggtgtggggaccataacatttatgttctgatatttgaaggactgtcaagtggaagaacaaaagttgcaattctcttctgctccagacatcagaaaaagattaaatttaatcttatatggagttatatcttagctcaatatgaaatgtaacattaaaataatgtttctatccaggtatccagctataaaaggggcttacataaaagcagagttttataaagtatcaatcaagttagtctagtttgtgctgtagcaacaaagaacccccaaatctcaatggtatatcaaaaaaagtttgtttcttatttatactactttatttgtccagcacaggtcacaaaagatcctacgcattgtagccttcaaagactcaagatgacagaagatccaccatcctatgacactgccatctaaacacaagtctccagcggccactgtggcaaggaaacagagcttgaatcataaatcagctcttaaatgcttctgcctggaagtgattcacatcacttcacttaaatttcattggccaaagcagtccatggccatgtataatttcaaggagatgagacagctgtaaaaggaaggatgtcagaagcttcagttagcacttggaacatctaccataactttcagtaggatttaagcagaattcaaattctcattaggaatatcatagaaaaagttagattgctaagcctctttaaactctaggattctataattccaaacttatgtcagatagttcctttaatatcagggattttgcttcctagggtaaaatgaataactctggagcactgaaacttcccatatacaaaggactatgctcaatatttgaatttactgagctgagcttacaaagacttggcttggaagagctaaatattggcaggtcaacagccctaactctgtaagcttgttatggtccatttttttcaaacattgcttcaaatatttacatttgacttttacataaaagttgctgattttcagtagaggctgagatgaacgacagttgataactgttcctcatgttctatagaatttatgtgtaaggtttccagctatttttctatcttccttggtaagactgtagtgtagctaaacaggtggacttaaatgtcagctgtattctagtggcttaataatgcctttgaatacgtaatagccaatgcttacaggttatgttattttatattacagtctcctgtttaattttactgcagatacgtcttaaattgagagcaattactcccttcatttttgccattttaaacctgctgtgtactcattttttttaaattatgggccaaaaaaggacagctatacattttcagtgtcatggatctagagttatagctctagaggggccacagagatcacctagtttgcccctttgttttacatacaaaaaatttaagaacagttaacatttgttgagagtgtaccatgttctgggcactggcctactgttttctcatgtattaactcaactgatcttctcaatagcccaagaaaataaatactgtcatcatctccatttcacagatgaataaacttacctaagattgggaaacatttcccccttattagacaggtcaatattttaaaaaaaaaaatggcatagcctggtgctggggagaacacgaacaggcacatggcctcatttactgttcagcattttgtgacatttagctcaaactttttgatattgaatcttcctccatttctccacagttcttacatatcaatttggacaaaggtgacaagataatagcaaattccaagaaaaactattacatagttcaaataatcacacaattacatattagacagaaagtaaaggctagagaaagtctgcagcactacctaatctgagaaaatgattgggaaggaatgttaaaattattaaccattgaggcttgggccctaggctcccttactgggaagtttctggaatagtttctagagttatgtctgaaatagttttccaattctgattgaaacctttaagctaataatgcttacctatgaatgaagagatttgggtgacttttacatttttctttgtacttttcaatattgtttaattttccattgcagtgacaatacattttataaaatcatcgagaagatttaaacaaatgcaatgagtttattgaatgagctgaactcaggaagatagcaaaaagcaactttgttctttctcaccctgtacctgcatacctgttctttgggtttcatttaacaagctattctacaacctaagagataggcactaccctcccactcctgaggtctaccacttttagaactgtctactattgtcaacactacctgcgacccagtcttcggcatcccctcctcaaactcatccccctaaagttccagtctctgtcctgctcagacacctgtgtcagggctctctccagtgattctgaattgagtgcccttgggcacccctggtaagagcctctgtctactcaaccacacccagagctaccattcgctgtatgaagctggaaaagttcacaccccttagctctggtgctgaagtggacacgggtagagcacaggaaaatgtgctccctacatcccaaatgaaagccctgaactaatagaaacaaatgatgaggaggctctgtatcactgaagtatggacacattgtgggttaaaggctttggcagactgaactggagacataaccttcattcatcacacaatttctatagaaaaatgtgtcgagttcaaaacaactgacctacaaatgatccttaggaacataatttgtctggaaactgggggctgcttttataaccatctccagcctgtcagatccaatagattagagtcaagacagcacctttgatttacagtcttggccctgttgctgaagcacttcctaattcacactctctattcttaaaatgagaggcataatatgtctgctccaactacaaggttgttgagataataagcatggctatttctgagaaaatatcttacaaaattgacaatataagtgtttactattatttcatgtggtgcattacagaattcacagtacaggtaattggttatagggaagtcgtttctgagattaataagactgccgcaaaagtatcacaatatgctcctgttttttccccattcctgatttctttccttagcaaaaaatgttcctttgtctttcttaacctatgcatttttaggttattggcttttagaatattggcattactgaaaccctgtctaactttaggagcgctaattgagtatataataacacacatgtaaatcaacaaattttagaaagccttagaatctgcaaaaagcatgaaacataatttatcctatgctaagtacagtaactaggtaatgccagtgttaaaaaaaaaagtataaaacttgaaaataaggataaaagggtagagcaagcccttttgatgtctactggtatattatttcaatagtccacttcatgacaatttatctgattactcatgtttgactttgctatttcctatttgattagagactagacactatggaattatatgttaaattgtagatttttgttaagtaaaaaagataaccttaaagatggctgttctgttgtcccgtgggccactaaccaatgttgtatccaacccagctatcctattctaatatccttttaatgtctttcctgctgtactatatatatcattgttccttaaatgctcttggaaccagtttcatcctcatattggtatgtatgtatatgtatacatatatacacatatatgtatatatgtatacattatctgtaaacataataaagtgctttgaagaaattttaaaaataggaaagtgggtggtgccaaggaagctgagggaagaaaatgtttgagaagggaatgctcagaagaggctgcactgccataagttgaagggacttagcagtaaggaataggtcagtaaccttggagagagcagcattcatggggtggtgaaggcagaaaccgcatcattaagagcaaggggaagagggccagaacgtacacaccactttagggaagttggaatgtggggagagcagtgcaatgagatggtgccagatagataagagatccaaggagaggtatatattttgtgtgttttctgggttttttgatgttgtttgttttaatgggtgagaccagagtatatttaaatgcagatgggaagaacagtttgaagatcaagtaagagggatggaggtgggggtgaataattaaaagaaaaaagattcctgaggaggcaagaggggatagaatcccaagaacagatatttcagggtgggggcggggctggcaacagacagcatgttggctggctgaagttacggtgggaggtggtgggagttgtaagtctgaggagcttgtgaaatgtttcagatggaagctgtgggaaatagaagaaagctaaaaaacacacatgaattgcaaaatagcattgaggaccccagtacaagttgaatgcaatgacatcatagtggcaccaatatgattatatgaggtttttttttctccagccatgctcaagacttcagcttagccaaggaaatagcaggcacggtaggtattttctggctggttatgagtggaatataatgagagaaggtaaataggacacttatagggaggtaactgaagcaatggactaagcacttgtccaaacatttttgttctcatgctctcaaaagattttggaaaactatttctcacatattttgaaatcaaaatctaaaaatttttaacacataaagtgaaatagtttcaaaggatgtatttatggcttatattatatatgtacattaaatatatttttatccaagtcttggagttgtagatttagctcattctatttatagaacacgtctttcagataatcaggccacattgtgaaactaatcagccaaatcagggttacttttcatcagaaccagtacaattttattttaaaattcatacagtcatgcatctgtggaatacttctgtattctaagataggttaattgatttttaaatggatggttgattgttgggtagatagctggtggatagatgaataaaacaagacatggatggatagacaaattcttatcttgagtttgtctcctggataaaacaagatcccctcaaatatttctctctgaagtttttttttattttactttcaagagactttccctcaagaaagtggtattctagatttgtccctctttttgatgccccaagtgtttttacaccctggagcaatgcatcaaaatacaacttaggatgggggaagtacacttttcttttgtaaagtggagaagggcaatgtgaaaggtgaaaaaggaaagactaattggtagacatcagagtttgtatgcaggtcagcttgaagaatgaatatgaggaagttgagatttagaaatttctacactacagctttctaagcttttttgattatcccacaggtacctaaaacttaacatgcctaaaattgaacttacatatctacctcatcctagtcctccttcctcagtgagtggcaccatttctattcattaagacaagacagaaacctggcagtcaccctgaacttcttgttctctcatgcccttcatatccaactaaacaccaagatctggacattttttctcataatgatctcctgagtcagcccacatccctctatccccatggctatctctctgctgcagggtatggttgcctctcactcagctgccaaaatctgcctgtctctagtcttgagtcctctccacctgctctccatactacaaccagagaaagtattctaaaacatgtctgactaaatagctccatttttaaaaagttatcaatgacttcctataaccctaggccttattattcacttactagattactatttcaatcaagctctaaggacaaatcctaaactcattggcatggctttcaaggcccttctgaacttggcctctgctcatcatggcagcttccgctctccccactccatactctgcttatgaagtgttttcatcccaagtctcaccaggctctcctgcctcaaacactctttctgcctccttcttctagctccctcctatttagcattaaggtttcagctgagatgtaatttcctctagaaagcttttcctaatccctcaagtttgggtttgatccttatcttacatacttctgtgacgcattgtttgtagtccattatagcatttactctacattgagttttaactgtttacatgtctgaatacccaagagcagagggacatatgtgtgtgtctattcacttttgtattgtcagtgtctagggtactagccactgcctggtgcagagtaggtatccaataaacacgtacttaccgaataaatacgtgaagctaccaaaattttgcccccaaaataaatcacattccttctatgagtggcttataaacctgtttagtgaccaaatataaagttttcatcaagttcatatgaaattgttggcaaaaaataatccataagcttgatggggaaaaaattccatgccccatctctctaacaatgatatcaaaaactacttccttatacatagcaaaataacttagctgagaactgagtcaaaaggaactgaaattttcattattttattaattcattcaatgatcaatggtcacttagctctgccttcatgaagcagtgttgctctagtctagtctaatgcttgccccatgaagcccactgaaccctggagaaaagctggcccatctcttcagctttccaaattttattatatagaactaggagcagctgcttttatccaagtaggaataatttttaaatagcatttttccttgtatgtcagaaaacccaagctgaaaatattacatttcttaaaacttctatgctcctgatctttttcttcttttctgttgtgccagaggcatgaactttatgcccccagcaccagttaagaagatgatttattaaacagacttaaatgaaagatggcttggtgtggatacacttagattcacagaccgtgccttggggcagttttagtgccaactttctaactaattcagaaatgaaaaacttctcattatttcaggataaatgtctaaacctaccagctcttgtctgaatgacataaaagtatcagcactaaaaatggagattttgttgttcacatgtcatctagactctcaaccctacaatgtttaacatatgagccagttacaaattaccaactaatggtatcttttgggcacttccaggtaaagcctcccagtgtccattgtatcaaactctttccctttcatacagggttacctgtacagtagtatcactcagaagttatgctggaggaattgctttcaattttttcattaggttcataaaatctactcagaaaatagatttaaaacacaaatgttaaaatccatgcaaaaacacaaatattttgatttgatttatgcaaagccctaagcctgtgctgtgcacagagaagagagcaatggcatgactacttgtctgtttactctcagaatgtgcatatatgcatttcatttccttgatttgaccctaattcaaggggccagtctgaagagtcagcaatgttaatttactagatctcaaaagtaagtattcatattactgcaaaaagcaagatgtcattttctcatcatttctgtgaatagaaaagctattttccaacaatagggatcccttataatagggaaatacttaactggtactgaactcagaaactgcagtgttctgcttggcttcattgattttatcaaaggacctctttatcctgagcaggtaaagctcaatgaattgaaatagtccagaaatacatgaatagctgtcctctgacagaaagtaagtttaaattgtaagaaaattactttatttccaaggattcccgagattcttgttcctgattatggtccaaaattccacacagatttgttcttgattcatttcagagtagtcagaaaaggtactgttctccttacatagagaaagaacatcctgtggtttcatctcagaactgtagctctcatatttgcaacagaaaaaagctggaccaacagcacactaatggctttttgtgaacccatcagaaagctaaagtcgaaggataatagtcttcctgaaatctagagagatgtggggtacctatgtaaaaattagagggctgtggtggacacaggaatcataaaatcagccagtccttttgctgaaatacatttctagtagtgccatgggtgatttgaaaatagtcttgttccttttcttcattcccttgcacactctgtctcctcttctccatggctttataaattacacacagaattaaggcttcccatttaggagaacatccatttctctctgacaacgtcatcaaagaagtgttcttcttccaagattttctcttgatgcagggaagtggcaaagttctagaagatcatcaagggctggaaatattgctgtggtcattccagagaaatgcaatagatgtgactgggcgcagcggccaccgtaaggcgtaaggggtgccaagtgccggttccagtcccgcccag

SEQ ID NO: 18799 - RNA, 13250 nt, Homo sapiens
  source 1..13250: mol_type = other RNA
tgatggataaaagactacatattgggtacagtgtactctgctagggtcatgggtacatcaaaatctcagaaatcaccactaaagaacttatccatgtaagcaaacaccacctgttccccaaaaactattgaaataaaaaataataacaataaatatctttaaaaatatgactctatttaaatgttgagataaaatgaggctctattttccacgaagaaattaataatgctaaaattaagaattccagtttctccaataaacaattatatatttaacaaaaagtagtttattaatcacctttgttattgctgatatttatcccattgatttagaatcactactgccttcctgagagctaaacatctctttaatcaaataacatttttattttttgcttattatttgaacatgtgccttaaaagcactgcctattttgtttctaataagatatttatttttacctattttttacattgcagatttgttccactgttgttgttgtttttgtttcaggtatagaatgccacatactacataaaatgattctttttgcttatgaataatgtcaccaatttttaaaataacttgcagaaaacaaaactatgactaggcgttttcagtaaaaatgctaacattttggcaactttgtgaaattgtttattcctcctgatggtgtatacaacagagaaatgtggagaaaatgttctactaagaactcaatgataatttgctctacctatcacattttttaaattccatgtggttgtctccattaacggatggttaaacagctccaatttgaagacaaaatctttgattttttaggaaacaaatttttggagtatcagataatcattagttttcttatgacttgcaaaaaatttaccttggttatagtggtagctagggtcagacagattaattatattaaggctagacagtactatttttgaaggtagtttctcttcccttttaatagtaatgaattatttaaacaggaatcatgtaactaacacttagcactgttctaagaactttccgtatattacctcaattaattatcatgtaaatccagcaagttaataacttttaaaactcctattttacagataaacaatttgtagcacaaagagataaacagcttgcccaaagtcacacagctaggaagggggatcccagaattaaaactcaagcattctgcacttaaaattactacacaatactggcccactagcttaccatgttccatggcagaatccaatcattttacccacggccattctttaataatggcttcgaacttcttactccatgacctttgctgcttattttctcatgcacaccacagaccacactggactcattccttccacaagaactctgccccttgaatagagaagagcttttaaaatcgtaagtcaggactcacatcttctctataatattctccctaagtgtagtaaaccattgaaatgttcaatattatatgcctattctaattacttggagtagttgtcaataatacagtattgagaaatatcttgagaaaaaaaactagccttactagataagtgcttgatcattagcaacttttgttctgaccacagaacaactcatagcaagctgtaagtttgttccccctgctactgaaaccaatgccaaagtatgaaatatgttaccttgctcctaaaagcaatgagacataaaatagttggcttaataataacattaaaaaattctatttaaaagcaagctatacttcattatccccatcttctgatttaatatattagataggcatttatctataaacttacttgatcaaatatttgagtgaccatgatacccaaggcactgtgctggtactgcagagaatacagggccgaggaaatgatcttgtactcaagtatagaaagcagaacactttttttttttgtgaagatatgatggttacagtagtatgactgttagatgcatgaactcagataggacagacatacaatcaaccacataaggcagaaactgataaatactaaaagaaaaaaaaacaaatattaggcagaaatgtggaatattattgaatcatatattcaaatataataattaaaataaatctaacataagaataagaatgtgagaggatgcaatgtgggaaactacttaaagcttgaggagataacatgtatcaataatgtgaacaagagcatggagggaagcccaagccaaagaaagcaataagcactgcatgggcaaggagaatcaggaagggaagctcccccagcctgcagcagagtggtgcctaactagtgatttgtgaagatggctaaaaggaggaggtgtgctgtgagagggcagcgcaggcacaggcacttgcaccatcaatgacatcttgaccctacagagccaaatggagatgggcgtccagctcccaggaggtggatttgtggatctaagcctcatgttacttctcagctgaattgaaagaaacagctacaaatccccaaagtacaaagagatgctaagcaagaacaggtgttcttgtggccagagcatcaaaagcaacacgtacctgtcatgtcccacttgaggagaaactagttctacttgtatgcaagtatgtgagtgataaatacataaatggttatgaatgctaacaaagtgctgtttattggaatttggagtctcagaaattggctcttcactcaaagatttcaaaataatgcactcctgcttttagttagcattaactatattttttatcagttggaaaatagctacctatgtaatagagaacatcgaactgaagaaaaccagagaagacttcataaaggaaagttctctcccattttctccctcctgctaaactgctccaacccctttctcactttcttccaaaatacaaatgtcctcctaaacagccctcttttctgagttgcagatcaaatgtctggaaatcctccatctgcaggtgacaatgttgaaagatctagcaaggccttctcctcctgcaacattccatatatgaactaatgatatcaccacttctctgctgccatttctaaaccacaaggcttgcccagggcctctcaaaacccactgtccatgactgtatctccacttattttcccttagctaaaaatgtgttctcccctgaactgctttccctgtgccccttgtatcaaggttgctcattcttttcatcctcatatatttaagggtaaggagttcatatcagtgtcttcttcattccccatagtaccttctcaatcattcccaccccaatgtgtttgtaaaaatctatacctctctgaatctggtcccatttttctgtacaacttattgtggacatctgtgagttaccaacacagcattcattctatcatgtgcccttgttaactatacttcaatttttttcaacagtgacccatccccctacttatgccctaaagtcaactttttgataaactgactttagttctacctctagaattagtgtatgcatttacctggccacattgatggccttaggcataatcttatcagagtgaagctcaaaacttttgttcagtggttgcaggaaatggacactttttcttccacgagaggcaaactaggaagaatggattcaccattgctgctgatacctgtcttgcaaccaggaggaaaatcagcctaaagaaaaaactaacatataaaggaaagaagaaccaaagaaacaggaaaaaagaaaatgtagaaccaagacctgattgaatagttcctgaaacaactttacttgtggacttttctgtttgtctttaagtcacttgagatgggttttctgtactttcattgactttgtcatcactagaaactgttccttttcaaattcctactttaaaaatcctatcctcagacatcagcctcctgtcctttcagtttgttcacttacacatactacagtactaattagaatgtcatatctgttgaccatttttactatccacctactccttcctattttcatatataagttttgttcaccagtgggccaacccatgtagctcagtgtcttacatttagtaggcaattaataaattgtgttgattcattggttaattgattgttctctttgcctttctctctcaccccttcccaagtatgcttcacctagtgattattcttttaaattttttccataattatttttctgtaacacaatatatccttattactgtcccactggaaatcttcaataacactcattttgtccatagctggacctcagatgtggtccacactatgttcctgatgttgttgctttctaaaggttatcatcttccaattgagattgaggatggacaaacccttcctgaaccaaattcagtgctggaagccaccttaaaatgtcaacttcaaatatggtctaaaataatgtacttttaataaataaatataactctccatcatcacaaacctcagaaaagccatgcaatgatctctcctgcagtatctaattttgtaagaattccattctagacattatgctttaatggaacactggcaaaataaaagttatccaaagagtaaccaggatggtgaaaagcccagaaaccatgtgtcaaggggaaaacagggtttctttgcagagagagggtgtggggaccataacatttatgttctgatatttgaaggactgtcaagtggaagaacaaaagttgcaattctcttctgctccagacatcagaaaaagattaaatttaatcttatatggagttatatcttagctcaatatgaaatgtaacattaaaataatgtttctatccaggtatccagctataaaaggggcttacataaaagcagagttttataaagtatcaatcaagttagtctagtttgtgctgtagcaacaaagaacccccaaatctcaatggtatatcaaaaaaagtttgtttcttatttatactactttatttgtccagcacaggtcacaaaagatcctacgcattgtagccttcaaagactcaagatgacagaagatccaccatcctatgacactgccatctaaacacaagtctccagcggccactgtggcaaggaaacagagcttgaatcataaatcagctcttaaatgcttctgcctggaagtgattcacatcacttcacttaaatttcattggccaaagcagtccatggccatgtataatttcaaggagatgagacagctgtaaaaggaaggatgtcagaagcttcagttagcacttggaacatctaccataactttcagtaggatttaagcagaattcaaattctcattaggaatatcatagaaaaagttagattgctaagcctctttaaactctaggattctataattccaaacttatgtcagatagttcctttaatatcagggattttgcttcctagggtaaaatgaataactctggagcactgaaacttcccatatacaaaggactatgctcaatatttgaatttactgagctgagcttacaaagacttggcttggaagagctaaatattggcaggtcaacagccctaactctgtaagcttgttatggtccatttttttcaaacattgcttcaaatatttacatttgacttttacataaaagttgctgattttcagtagaggctgagatgaacgacagttgataactgttcctcatgttctatagaatttatgtgtaaggtttccagctatttttctatcttccttggtaagactgtagtgtagctaaacaggtggacttaaatgtcagctgtattctagtggcttaataatgcctttgaatacgtaatagccaatgcttacaggttatgttattttatattacagtctcctgtttaattttactgcagatacgtcttaaattgagagcaattactcccttcatttttgccattttaaacctgctgtgtactcattttttttaaattatgggccaaaaaaggacagctatacattttcagtgtcatggatctagagttatagctctagaggggccacagagatcacctagtttgcccctttgttttacatacaaaaaatttaagaacagttaacatttgttgagagtgtaccatgttctgggcactggcctactgttttctcatgtattaactcaactgatcttctcaatagcccaagaaaataaatactgtcatcatctccatttcacagatgaataaacttacctaagattgggaaacatttcccccttattagacaggtcaatattttaaaaaaaaaaatggcatagcctggtgctggggagaacacgaacaggcacatggcctcatttactgttcagcattttgtgacatttagctcaaactttttgatattgaatcttcctccatttctccacagttcttacatatcaatttggacaaaggtgacaagataatagcaaattccaagaaaaactattacatagttcaaataatcacacaattacatattagacagaaagtaaaggctagagaaagtctgcagcactacctaatctgagaaaatgattgggaaggaatgttaaaattattaaccattgaggcttgggccctaggctcccttactgggaagtttctggaatagtttctagagttatgtctgaaatagttttccaattctgattgaaacctttaagctaataatgcttacctatgaatgaagagatttgggtgacttttacatttttctttgtacttttcaatattgtttaattttccattgcagtgacaatacattttataaaatcatcgagaagatttaaacaaatgcaatgagtttattgaatgagctgaactcaggaagatagcaaaaagcaactttgttctttctcaccctgtacctgcatacctgttctttgggtttcatttaacaagctattctacaacctaagagataggcactaccctcccactcctgaggtctaccacttttagaactgtctactattgtcaacactacctgcgacccagtcttcggcatcccctcctcaaactcatccccctaaagttccagtctctgtcctgctcagacacctgtgtcagggctctctccagtgattctgaattgagtgcccttgggcacccctggtaagagcctctgtctactcaaccacacccagagctaccattcgctgtatgaagctggaaaagttcacaccccttagctctggtgctgaagtggacacgggtagagcacaggaaaatgtgctccctacatcccaaatgaaagccctgaactaatagaaacaaatgatgaggaggctctgtatcactgaagtatggacacattgtgggttaaaggctttggcagactgaactggagacataaccttcattcatcacacaatttctatagaaaaatgtgtcgagttcaaaacaactgacctacaaatgatccttaggaacataatttgtctggaaactgggggctgcttttataaccatctccagcctgtcagatccaatagattagagtcaagacagcacctttgatttacagtcttggccctgttgctgaagcacttcctaattcacactctctattcttaaaatgagaggcataatatgtctgctccaactacaaggttgttgagataataagcatggctatttctgagaaaatatcttacaaaattgacaatataagtgtttactattatttcatgtggtgcattacagaattcacagtacaggtaattggttatagggaagtcgtttctgagattaataagactgccgcaaaagtatcacaatatgctcctgttttttccccattcctgatttctttccttagcaaaaaatgttcctttgtctttcttaacctatgcatttttaggttattggcttttagaatattggcattactgaaaccctgtctaactttaggagcgctaattgagtatataataacacacatgtaaatcaacaaattttagaaagccttagaatctgcaaaaagcatgaaacataatttatcctatgctaagtacagtaactaggtaatgccagtgttaaaaaaaaaagtataaaacttgaaaataaggataaaagggtagagcaagcccttttgatgtctactggtatattatttcaatagtccacttcatgacaatttatctgattactcatgtttgactttgctatttcctatttgattagagactagacactatggaattatatgttaaattgtagatttttgttaagtaaaaaagataaccttaaagatggctgttctgttgtcccgtgggccactaaccaatgttgtatccaacccagctatcctattctaatatccttttaatgtctttcctgctgtactatatatatcattgttccttaaatgctcttggaaccagtttcatcctcatattggtatgtatgtatatgtatacatatatacacatatatgtatatatgtatacattatctgtaaacataataaagtgctttgaagaaattttaaaaataggaaagtgggtggtgccaaggaagctgagggaagaaaatgtttgagaagggaatgctcagaagaggctgcactgccataagttgaagggacttagcagtaaggaataggtcagtaaccttggagagagcagcattcatggggtggtgaaggcagaaaccgcatcattaagagcaaggggaagagggccagaacgtacacaccactttagggaagttggaatgtggggagagcagtgcaatgagatggtgccagatagataagagatccaaggagaggtatatattttgtgtgttttctgggttttttgatgttgtttgttttaatgggtgagaccagagtatatttaaatgcagatgggaagaacagtttgaagatcaagtaagagggatggaggtgggggtgaataattaaaagaaaaaagattcctgaggaggcaagaggggatagaatcccaagaacagatatttcagggtgggggcggggctggcaacagacagcatgttggctggctgaagttacggtgggaggtggtgggagttgtaagtctgaggagcttgtgaaatgtttcagatggaagctgtgggaaatagaagaaagctaaaaaacacacatgaattgcaaaatagcattgaggaccccagtacaagttgaatgcaatgacatcatagtggcaccaatatgattatatgaggtttttttttctccagccatgctcaagacttcagcttagccaaggaaatagcaggcacggtaggtattttctggctggttatgagtggaatataatgagagaaggtaaataggacacttatagggaggtaactgaagcaatggactaagcacttgtccaaacatttttgttctcatgctctcaaaagattttggaaaactatttctcacatattttgaaatcaaaatctaaaaatttttaacacataaagtgaaatagtttcaaaggatgtatttatggcttatattatatatgtacattaaatatatttttatccaagtcttggagttgtagatttagctcattctatttatagaacacgtctttcagataatcaggccacattgtgaaactaatcagccaaatcagggttacttttcatcagaaccagtacaattttattttaaaattcatacagtcatgcatctgtggaatacttctgtattctaagataggttaattgatttttaaatggatggttgattgttgggtagatagctggtggatagatgaataaaacaagacatggatggatagacaaattcttatcttgagtttgtctcctggataaaacaagatcccctcaaatatttctctctgaagtttttttttattttactttcaagagactttccctcaagaaagtggtattctagatttgtccctctttttgatgccccaagtgtttttacaccctggagcaatgcatcaaaatacaacttaggatgggggaagtacacttttcttttgtaaagtggagaagggcaatgtgaaaggtgaaaaaggaaagactaattggtagacatcagagtttgtatgcaggtcagcttgaagaatgaatatgaggaagttgagatttagaaatttctacactacagctttctaagcttttttgattatcccacaggtacctaaaacttaacatgcctaaaattgaacttacatatctacctcatcctagtcctccttcctcagtgagtggcaccatttctattcattaagacaagacagaaacctggcagtcaccctgaacttcttgttctctcatgcccttcatatccaactaaacaccaagatctggacattttttctcataatgatctcctgagtcagcccacatccctctatccccatggctatctctctgctgcagggtatggttgcctctcactcagctgccaaaatctgcctgtctctagtcttgagtcctctccacctgctctccatactacaaccagagaaagtattctaaaacatgtctgactaaatagctccatttttaaaaagttatcaatgacttcctataaccctaggccttattattcacttactagattactatttcaatcaagctctaaggacaaatcctaaactcattggcatggctttcaaggcccttctgaacttggcctctgctcatcatggcagcttccgctctccccactccatactctgcttatgaagtgttttcatcccaagtctcaccaggctctcctgcctcaaacactctttctgcctccttcttctagctccctcctatttagcattaaggtttcagctgagatgtaatttcctctagaaagcttttcctaatccctcaagtttgggtttgatccttatcttacatacttctgtgacgcattgtttgtagtccattatagcatttactctacattgagttttaactgtttacatgtctgaatacccaagagcagagggacatatgtgtgtgtctattcacttttgtattgtcagtgtctagggtactagccactgcctggtgcagagtaggtatccaataaacacgtacttaccgaataaatacgtgaagctaccaaaattttgcccccaaaataaatcacattccttctatgagtggcttataaacctgtttagtgaccaaatataaagttttcatcaagttcatatgaaattgttggcaaaaaataatccataagcttgatggggaaaaaattccatgccccatctctctaacaatgatatcaaaaactacttccttatacatagcaaaataacttagctgagaactgagtcaaaaggaactgaaattttcattattttattaattcattcaatgatcaatggtcacttagctctgccttcatgaagcagtgttgctctagtctagtctaatgcttgccccatgaagcccactgaaccctggagaaaagctggcccatctcttcagctttccaaattttattatatagaactaggagcagctgcttttatccaagtaggaataatttttaaatagcatttttccttgtatgtcagaaaacccaagctgaaaatattacatttcttaaaacttctatgctcctgatctttttcttcttttctgttgtgccagaggcatgaactttatgcccccagcaccagttaagaagatgatttattaaacagacttaaatgaaagatggcttggtgtggatacacttagattcacagaccgtgccttggggcagttttagtgccaactttctaactaattcagaaatgaaaaacttctcattatttcaggataaatgtctaaacctaccagctcttgtctgaatgacataaaagtatcagcactaaaaatggagattttgttgttcacatgtcatctagactctcaaccctacaatgtttaacatatgagccagttacaaattaccaactaatggtatcttttgggcacttccaggtaaagcctcccagtgtccattgtatcaaactctttccctttcatacagggttacctgtacagtagtatcactcagaagttatgctggaggaattgctttcaattttttcattaggttcataaaatctactcagaaaatagatttaaaacacaaatgttaaaatccatgcaaaaacacaaatattttgatttgatttatgcaaagccctaagcctgtgctgtgcacagagaagagagcaatggcatgactacttgtctgtttactctcagaatgtgcatatatgcatttcatttccttgatttgaccctaattcaaggggccagtctgaagagtcagcaatgttaatttactagatctcaaaagtaagtattcatattactgcaaaaagcaagatgtcattttctcatcatttctgtgaatagaaaagctattttccaacaatagggatcccttataatagggaaatacttaactggtactgaactcagaaactgcagtgttctgcttggcttcattgattttatcaaaggacctctttatcctgagcaggtaaagctcaatgaattgaaatagtccagaaatacatgaatagctgtcctctgacagaaagtaagtttaaattgtaagaaaattactttatttccaaggattcccgagattcttgttcctgattatggtccaaaattccacacagatttgttcttgattcatttcagagtagtcagaaaaggtactgttctccttacatagagaaagaacatcctgtggtttcatctcagaactgtagctctcatatttgcaacagaaaaaagctggaccaacagcacactaatggctttttgtgaacccatcagaaagctaaagtcgaaggataatagtcttcctgaaatctagagagatgtggggtacctatgtaaaaattagagggctgtggtggacacaggaatcataaaatcagccagtccttttgctgaaatacatttctagtagtgccatgggtgatttgaaaatagtcttgttccttttcttcattcccttgcacactctgtctcctcttctccatggctttataaattacacacagaattaaggcttcccatttaggagaacatccatttctctctgacaacgtcatcaaagaagtgttcttcttccaagattttctcttgatgcagggaagtggcaaagttctagaagatcatcaagggctggaaatattgctgtggtcattccagagaaatgcaataggcaatcgggcgctcccctcttccggaagtcgcgccggtgcgcgccggactcctcccaccagcggcgacgtcaaactcag

SEQ ID NO: 18800 - RNA, 13252 nt, Homo sapiens
  source 1..13252: mol_type = other RNA
tgatggataaaagactacatattgggtacagtgtactctgctagggtcatgggtacatcaaaatctcagaaatcaccactaaagaacttatccatgtaagcaaacaccacctgttccccaaaaactattgaaataaaaaataataacaataaatatctttaaaaatatgactctatttaaatgttgagataaaatgaggctctattttccacgaagaaattaataatgctaaaattaagaattccagtttctccaataaacaattatatatttaacaaaaagtagtttattaatcacctttgttattgctgatatttatcccattgatttagaatcactactgccttcctgagagctaaacatctctttaatcaaataacatttttattttttgcttattatttgaacatgtgccttaaaagcactgcctattttgtttctaataagatatttatttttacctattttttacattgcagatttgttccactgttgttgttgtttttgtttcaggtatagaatgccacatactacataaaatgattctttttgcttatgaataatgtcaccaatttttaaaataacttgcagaaaacaaaactatgactaggcgttttcagtaaaaatgctaacattttggcaactttgtgaaattgtttattcctcctgatggtgtatacaacagagaaatgtggagaaaatgttctactaagaactcaatgataatttgctctacctatcacattttttaaattccatgtggttgtctccattaacggatggttaaacagctccaatttgaagacaaaatctttgattttttaggaaacaaatttttggagtatcagataatcattagttttcttatgacttgcaaaaaatttaccttggttatagtggtagctagggtcagacagattaattatattaaggctagacagtactatttttgaaggtagtttctcttcccttttaatagtaatgaattatttaaacaggaatcatgtaactaacacttagcactgttctaagaactttccgtatattacctcaattaattatcatgtaaatccagcaagttaataacttttaaaactcctattttacagataaacaatttgtagcacaaagagataaacagcttgcccaaagtcacacagctaggaagggggatcccagaattaaaactcaagcattctgcacttaaaattactacacaatactggcccactagcttaccatgttccatggcagaatccaatcattttacccacggccattctttaataatggcttcgaacttcttactccatgacctttgctgcttattttctcatgcacaccacagaccacactggactcattccttccacaagaactctgccccttgaatagagaagagcttttaaaatcgtaagtcaggactcacatcttctctataatattctccctaagtgtagtaaaccattgaaatgttcaatattatatgcctattctaattacttggagtagttgtcaataatacagtattgagaaatatcttgagaaaaaaaactagccttactagataagtgcttgatcattagcaacttttgttctgaccacagaacaactcatagcaagctgtaagtttgttccccctgctactgaaaccaatgccaaagtatgaaatatgttaccttgctcctaaaagcaatgagacataaaatagttggcttaataataacattaaaaaattctatttaaaagcaagctatacttcattatccccatcttctgatttaatatattagataggcatttatctataaacttacttgatcaaatatttgagtgaccatgatacccaaggcactgtgctggtactgcagagaatacagggccgaggaaatgatcttgtactcaagtatagaaagcagaacactttttttttttgtgaagatatgatggttacagtagtatgactgttagatgcatgaactcagataggacagacatacaatcaaccacataaggcagaaactgataaatactaaaagaaaaaaaaacaaatattaggcagaaatgtggaatattattgaatcatatattcaaatataataattaaaataaatctaacataagaataagaatgtgagaggatgcaatgtgggaaactacttaaagcttgaggagataacatgtatcaataatgtgaacaagagcatggagggaagcccaagccaaagaaagcaataagcactgcatgggcaaggagaatcaggaagggaagctcccccagcctgcagcagagtggtgcctaactagtgatttgtgaagatggctaaaaggaggaggtgtgctgtgagagggcagcgcaggcacaggcacttgcaccatcaatgacatcttgaccctacagagccaaatggagatgggcgtccagctcccaggaggtggatttgtggatctaagcctcatgttacttctcagctgaattgaaagaaacagctacaaatccccaaagtacaaagagatgctaagcaagaacaggtgttcttgtggccagagcatcaaaagcaacacgtacctgtcatgtcccacttgaggagaaactagttctacttgtatgcaagtatgtgagtgataaatacataaatggttatgaatgctaacaaagtgctgtttattggaatttggagtctcagaaattggctcttcactcaaagatttcaaaataatgcactcctgcttttagttagcattaactatattttttatcagttggaaaatagctacctatgtaatagagaacatcgaactgaagaaaaccagagaagacttcataaaggaaagttctctcccattttctccctcctgctaaactgctccaacccctttctcactttcttccaaaatacaaatgtcctcctaaacagccctcttttctgagttgcagatcaaatgtctggaaatcctccatctgcaggtgacaatgttgaaagatctagcaaggccttctcctcctgcaacattccatatatgaactaatgatatcaccacttctctgctgccatttctaaaccacaaggcttgcccagggcctctcaaaacccactgtccatgactgtatctccacttattttcccttagctaaaaatgtgttctcccctgaactgctttccctgtgccccttgtatcaaggttgctcattcttttcatcctcatatatttaagggtaaggagttcatatcagtgtcttcttcattccccatagtaccttctcaatcattcccaccccaatgtgtttgtaaaaatctatacctctctgaatctggtcccatttttctgtacaacttattgtggacatctgtgagttaccaacacagcattcattctatcatgtgcccttgttaactatacttcaatttttttcaacagtgacccatccccctacttatgccctaaagtcaactttttgataaactgactttagttctacctctagaattagtgtatgcatttacctggccacattgatggccttaggcataatcttatcagagtgaagctcaaaacttttgttcagtggttgcaggaaatggacactttttcttccacgagaggcaaactaggaagaatggattcaccattgctgctgatacctgtcttgcaaccaggaggaaaatcagcctaaagaaaaaactaacatataaaggaaagaagaaccaaagaaacaggaaaaaagaaaatgtagaaccaagacctgattgaatagttcctgaaacaactttacttgtggacttttctgtttgtctttaagtcacttgagatgggttttctgtactttcattgactttgtcatcactagaaactgttccttttcaaattcctactttaaaaatcctatcctcagacatcagcctcctgtcctttcagtttgttcacttacacatactacagtactaattagaatgtcatatctgttgaccatttttactatccacctactccttcctattttcatatataagttttgttcaccagtgggccaacccatgtagctcagtgtcttacatttagtaggcaattaataaattgtgttgattcattggttaattgattgttctctttgcctttctctctcaccccttcccaagtatgcttcacctagtgattattcttttaaattttttccataattatttttctgtaacacaatatatccttattactgtcccactggaaatcttcaataacactcattttgtccatagctggacctcagatgtggtccacactatgttcctgatgttgttgctttctaaaggttatcatcttccaattgagattgaggatggacaaacccttcctgaaccaaattcagtgctggaagccaccttaaaatgtcaacttcaaatatggtctaaaataatgtacttttaataaataaatataactctccatcatcacaaacctcagaaaagccatgcaatgatctctcctgcagtatctaattttgtaagaattccattctagacattatgctttaatggaacactggcaaaataaaagttatccaaagagtaaccaggatggtgaaaagcccagaaaccatgtgtcaaggggaaaacagggtttctttgcagagagagggtgtggggaccataacatttatgttctgatatttgaaggactgtcaagtggaagaacaaaagttgcaattctcttctgctccagacatcagaaaaagattaaatttaatcttatatggagttatatcttagctcaatatgaaatgtaacattaaaataatgtttctatccaggtatccagctataaaaggggcttacataaaagcagagttttataaagtatcaatcaagttagtctagtttgtgctgtagcaacaaagaacccccaaatctcaatggtatatcaaaaaaagtttgtttcttatttatactactttatttgtccagcacaggtcacaaaagatcctacgcattgtagccttcaaagactcaagatgacagaagatccaccatcctatgacactgccatctaaacacaagtctccagcggccactgtggcaaggaaacagagcttgaatcataaatcagctcttaaatgcttctgcctggaagtgattcacatcacttcacttaaatttcattggccaaagcagtccatggccatgtataatttcaaggagatgagacagctgtaaaaggaaggatgtcagaagcttcagttagcacttggaacatctaccataactttcagtaggatttaagcagaattcaaattctcattaggaatatcatagaaaaagttagattgctaagcctctttaaactctaggattctataattccaaacttatgtcagatagttcctttaatatcagggattttgcttcctagggtaaaatgaataactctggagcactgaaacttcccatatacaaaggactatgctcaatatttgaatttactgagctgagcttacaaagacttggcttggaagagctaaatattggcaggtcaacagccctaactctgtaagcttgttatggtccatttttttcaaacattgcttcaaatatttacatttgacttttacataaaagttgctgattttcagtagaggctgagatgaacgacagttgataactgttcctcatgttctatagaatttatgtgtaaggtttccagctatttttctatcttccttggtaagactgtagtgtagctaaacaggtggacttaaatgtcagctgtattctagtggcttaataatgcctttgaatacgtaatagccaatgcttacaggttatgttattttatattacagtctcctgtttaattttactgcagatacgtcttaaattgagagcaattactcccttcatttttgccattttaaacctgctgtgtactcattttttttaaattatgggccaaaaaaggacagctatacattttcagtgtcatggatctagagttatagctctagaggggccacagagatcacctagtttgcccctttgttttacatacaaaaaatttaagaacagttaacatttgttgagagtgtaccatgttctgggcactggcctactgttttctcatgtattaactcaactgatcttctcaatagcccaagaaaataaatactgtcatcatctccatttcacagatgaataaacttacctaagattgggaaacatttcccccttattagacaggtcaatattttaaaaaaaaaaatggcatagcctggtgctggggagaacacgaacaggcacatggcctcatttactgttcagcattttgtgacatttagctcaaactttttgatattgaatcttcctccatttctccacagttcttacatatcaatttggacaaaggtgacaagataatagcaaattccaagaaaaactattacatagttcaaataatcacacaattacatattagacagaaagtaaaggctagagaaagtctgcagcactacctaatctgagaaaatgattgggaaggaatgttaaaattattaaccattgaggcttgggccctaggctcccttactgggaagtttctggaatagtttctagagttatgtctgaaatagttttccaattctgattgaaacctttaagctaataatgcttacctatgaatgaagagatttgggtgacttttacatttttctttgtacttttcaatattgtttaattttccattgcagtgacaatacattttataaaatcatcgagaagatttaaacaaatgcaatgagtttattgaatgagctgaactcaggaagatagcaaaaagcaactttgttctttctcaccctgtacctgcatacctgttctttgggtttcatttaacaagctattctacaacctaagagataggcactaccctcccactcctgaggtctaccacttttagaactgtctactattgtcaacactacctgcgacccagtcttcggcatcccctcctcaaactcatccccctaaagttccagtctctgtcctgctcagacacctgtgtcagggctctctccagtgattctgaattgagtgcccttgggcacccctggtaagagcctctgtctactcaaccacacccagagctaccattcgctgtatgaagctggaaaagttcacaccccttagctctggtgctgaagtggacacgggtagagcacaggaaaatgtgctccctacatcccaaatgaaagccctgaactaatagaaacaaatgatgaggaggctctgtatcactgaagtatggacacattgtgggttaaaggctttggcagactgaactggagacataaccttcattcatcacacaatttctatagaaaaatgtgtcgagttcaaaacaactgacctacaaatgatccttaggaacataatttgtctggaaactgggggctgcttttataaccatctccagcctgtcagatccaatagattagagtcaagacagcacctttgatttacagtcttggccctgttgctgaagcacttcctaattcacactctctattcttaaaatgagaggcataatatgtctgctccaactacaaggttgttgagataataagcatggctatttctgagaaaatatcttacaaaattgacaatataagtgtttactattatttcatgtggtgcattacagaattcacagtacaggtaattggttatagggaagtcgtttctgagattaataagactgccgcaaaagtatcacaatatgctcctgttttttccccattcctgatttctttccttagcaaaaaatgttcctttgtctttcttaacctatgcatttttaggttattggcttttagaatattggcattactgaaaccctgtctaactttaggagcgctaattgagtatataataacacacatgtaaatcaacaaattttagaaagccttagaatctgcaaaaagcatgaaacataatttatcctatgctaagtacagtaactaggtaatgccagtgttaaaaaaaaaagtataaaacttgaaaataaggataaaagggtagagcaagcccttttgatgtctactggtatattatttcaatagtccacttcatgacaatttatctgattactcatgtttgactttgctatttcctatttgattagagactagacactatggaattatatgttaaattgtagatttttgttaagtaaaaaagataaccttaaagatggctgttctgttgtcccgtgggccactaaccaatgttgtatccaacccagctatcctattctaatatccttttaatgtctttcctgctgtactatatatatcattgttccttaaatgctcttggaaccagtttcatcctcatattggtatgtatgtatatgtatacatatatacacatatatgtatatatgtatacattatctgtaaacataataaagtgctttgaagaaattttaaaaataggaaagtgggtggtgccaaggaagctgagggaagaaaatgtttgagaagggaatgctcagaagaggctgcactgccataagttgaagggacttagcagtaaggaataggtcagtaaccttggagagagcagcattcatggggtggtgaaggcagaaaccgcatcattaagagcaaggggaagagggccagaacgtacacaccactttagggaagttggaatgtggggagagcagtgcaatgagatggtgccagatagataagagatccaaggagaggtatatattttgtgtgttttctgggttttttgatgttgtttgttttaatgggtgagaccagagtatatttaaatgcagatgggaagaacagtttgaagatcaagtaagagggatggaggtgggggtgaataattaaaagaaaaaagattcctgaggaggcaagaggggatagaatcccaagaacagatatttcagggtgggggcggggctggcaacagacagcatgttggctggctgaagttacggtgggaggtggtgggagttgtaagtctgaggagcttgtgaaatgtttcagatggaagctgtgggaaatagaagaaagctaaaaaacacacatgaattgcaaaatagcattgaggaccccagtacaagttgaatgcaatgacatcatagtggcaccaatatgattatatgaggtttttttttctccagccatgctcaagacttcagcttagccaaggaaatagcaggcacggtaggtattttctggctggttatgagtggaatataatgagagaaggtaaataggacacttatagggaggtaactgaagcaatggactaagcacttgtccaaacatttttgttctcatgctctcaaaagattttggaaaactatttctcacatattttgaaatcaaaatctaaaaatttttaacacataaagtgaaatagtttcaaaggatgtatttatggcttatattatatatgtacattaaatatatttttatccaagtcttggagttgtagatttagctcattctatttatagaacacgtctttcagataatcaggccacattgtgaaactaatcagccaaatcagggttacttttcatcagaaccagtacaattttattttaaaattcatacagtcatgcatctgtggaatacttctgtattctaagataggttaattgatttttaaatggatggttgattgttgggtagatagctggtggatagatgaataaaacaagacatggatggatagacaaattcttatcttgagtttgtctcctggataaaacaagatcccctcaaatatttctctctgaagtttttttttattttactttcaagagactttccctcaagaaagtggtattctagatttgtccctctttttgatgccccaagtgtttttacaccctggagcaatgcatcaaaatacaacttaggatgggggaagtacacttttcttttgtaaagtggagaagggcaatgtgaaaggtgaaaaaggaaagactaattggtagacatcagagtttgtatgcaggtcagcttgaagaatgaatatgaggaagttgagatttagaaatttctacactacagctttctaagcttttttgattatcccacaggtacctaaaacttaacatgcctaaaattgaacttacatatctacctcatcctagtcctccttcctcagtgagtggcaccatttctattcattaagacaagacagaaacctggcagtcaccctgaacttcttgttctctcatgcccttcatatccaactaaacaccaagatctggacattttttctcataatgatctcctgagtcagcccacatccctctatccccatggctatctctctgctgcagggtatggttgcctctcactcagctgccaaaatctgcctgtctctagtcttgagtcctctccacctgctctccatactacaaccagagaaagtattctaaaacatgtctgactaaatagctccatttttaaaaagttatcaatgacttcctataaccctaggccttattattcacttactagattactatttcaatcaagctctaaggacaaatcctaaactcattggcatggctttcaaggcccttctgaacttggcctctgctcatcatggcagcttccgctctccccactccatactctgcttatgaagtgttttcatcccaagtctcaccaggctctcctgcctcaaacactctttctgcctccttcttctagctccctcctatttagcattaaggtttcagctgagatgtaatttcctctagaaagcttttcctaatccctcaagtttgggtttgatccttatcttacatacttctgtgacgcattgtttgtagtccattatagcatttactctacattgagttttaactgtttacatgtctgaatacccaagagcagagggacatatgtgtgtgtctattcacttttgtattgtcagtgtctagggtactagccactgcctggtgcagagtaggtatccaataaacacgtacttaccgaataaatacgtgaagctaccaaaattttgcccccaaaataaatcacattccttctatgagtggcttataaacctgtttagtgaccaaatataaagttttcatcaagttcatatgaaattgttggcaaaaaataatccataagcttgatggggaaaaaattccatgccccatctctctaacaatgatatcaaaaactacttccttatacatagcaaaataacttagctgagaactgagtcaaaaggaactgaaattttcattattttattaattcattcaatgatcaatggtcacttagctctgccttcatgaagcagtgttgctctagtctagtctaatgcttgccccatgaagcccactgaaccctggagaaaagctggcccatctcttcagctttccaaattttattatatagaactaggagcagctgcttttatccaagtaggaataatttttaaatagcatttttccttgtatgtcagaaaacccaagctgaaaatattacatttcttaaaacttctatgctcctgatctttttcttcttttctgttgtgccagaggcatgaactttatgcccccagcaccagttaagaagatgatttattaaacagacttaaatgaaagatggcttggtgtggatacacttagattcacagaccgtgccttggggcagttttagtgccaactttctaactaattcagaaatgaaaaacttctcattatttcaggataaatgtctaaacctaccagctcttgtctgaatgacataaaagtatcagcactaaaaatggagattttgttgttcacatgtcatctagactctcaaccctacaatgtttaacatatgagccagttacaaattaccaactaatggtatcttttgggcacttccaggtaaagcctcccagtgtccattgtatcaaactctttccctttcatacagggttacctgtacagtagtatcactcagaagttatgctggaggaattgctttcaattttttcattaggttcataaaatctactcagaaaatagatttaaaacacaaatgttaaaatccatgcaaaaacacaaatattttgatttgatttatgcaaagccctaagcctgtgctgtgcacagagaagagagcaatggcatgactacttgtctgtttactctcagaatgtgcatatatgcatttcatttccttgatttgaccctaattcaaggggccagtctgaagagtcagcaatgttaatttactagatctcaaaagtaagtattcatattactgcaaaaagcaagatgtcattttctcatcatttctgtgaatagaaaagctattttccaacaatagggatcccttataatagggaaatacttaactggtactgaactcagaaactgcagtgttctgcttggcttcattgattttatcaaaggacctctttatcctgagcaggtaaagctcaatgaattgaaatagtccagaaatacatgaatagctgtcctctgacagaaagtaagtttaaattgtaagaaaattactttatttccaaggattcccgagattcttgttcctgattatggtccaaaattccacacagatttgttcttgattcatttcagagtagtcagaaaaggtactgttctccttacatagagaaagaacatcctgtggtttcatctcagaactgtagctctcatatttgcaacagaaaaaagctggaccaacagcacactaatggctttttgtgaacccatcagaaagctaaagtcgaaggataatagtcttcctgaaatctagagagatgtggggtacctatgtaaaaattagagggctgtggtggacacaggaatcataaaatcagccagtccttttgctgaaatacatttctagtagtgccatgggtgatttgaaaatagtcttgttccttttcttcattcccttgcacactctgtctcctcttctccatggctttataaattacacacagaattaaggcttcccatttaggagaacatccatttctctctgacaacgtcatcaaagaagtgttcttcttccaagattttctcttgatgcagggaagtggcaaagttctagaagatcatcaagggctggaaatattgctgtggtcattccagagaaatgcaatcacttctctgtctctgccgaccggcgcagggagggctgccttttccttacagtacgccttgaggcttccgggccgctgaagtt

SEQ ID NO: 18801 - RNA, 13597 nt, Homo sapiens
  source 1..13597: mol_type = other RNA
tgatggataaaagactacatattgggtacagtgtactctgctagggtcatgggtacatcaaaatctcagaaatcaccactaaagaacttatccatgtaagcaaacaccacctgttccccaaaaactattgaaataaaaaataataacaataaatatctttaaaaatatgactctatttaaatgttgagataaaatgaggctctattttccacgaagaaattaataatgctaaaattaagaattccagtttctccaataaacaattatatatttaacaaaaagtagtttattaatcacctttgttattgctgatatttatcccattgatttagaatcactactgccttcctgagagctaaacatctctttaatcaaataacatttttattttttgcttattatttgaacatgtgccttaaaagcactgcctattttgtttctaataagatatttatttttacctattttttacattgcagatttgttccactgttgttgttgtttttgtttcaggtatagaatgccacatactacataaaatgattctttttgcttatgaataatgtcaccaatttttaaaataacttgcagaaaacaaaactatgactaggcgttttcagtaaaaatgctaacattttggcaactttgtgaaattgtttattcctcctgatggtgtatacaacagagaaatgtggagaaaatgttctactaagaactcaatgataatttgctctacctatcacattttttaaattccatgtggttgtctccattaacggatggttaaacagctccaatttgaagacaaaatctttgattttttaggaaacaaatttttggagtatcagataatcattagttttcttatgacttgcaaaaaatttaccttggttatagtggtagctagggtcagacagattaattatattaaggctagacagtactatttttgaaggtagtttctcttcccttttaatagtaatgaattatttaaacaggaatcatgtaactaacacttagcactgttctaagaactttccgtatattacctcaattaattatcatgtaaatccagcaagttaataacttttaaaactcctattttacagataaacaatttgtagcacaaagagataaacagcttgcccaaagtcacacagctaggaagggggatcccagaattaaaactcaagcattctgcacttaaaattactacacaatactggcccactagcttaccatgttccatggcagaatccaatcattttacccacggccattctttaataatggcttcgaacttcttactccatgacctttgctgcttattttctcatgcacaccacagaccacactggactcattccttccacaagaactctgccccttgaatagagaagagcttttaaaatcgtaagtcaggactcacatcttctctataatattctccctaagtgtagtaaaccattgaaatgttcaatattatatgcctattctaattacttggagtagttgtcaataatacagtattgagaaatatcttgagaaaaaaaactagccttactagataagtgcttgatcattagcaacttttgttctgaccacagaacaactcatagcaagctgtaagtttgttccccctgctactgaaaccaatgccaaagtatgaaatatgttaccttgctcctaaaagcaatgagacataaaatagttggcttaataataacattaaaaaattctatttaaaagcaagctatacttcattatccccatcttctgatttaatatattagataggcatttatctataaacttacttgatcaaatatttgagtgaccatgatacccaaggcactgtgctggtactgcagagaatacagggccgaggaaatgatcttgtactcaagtatagaaagcagaacactttttttttttgtgaagatatgatggttacagtagtatgactgttagatgcatgaactcagataggacagacatacaatcaaccacataaggcagaaactgataaatactaaaagaaaaaaaaacaaatattaggcagaaatgtggaatattattgaatcatatattcaaatataataattaaaataaatctaacataagaataagaatgtgagaggatgcaatgtgggaaactacttaaagcttgaggagataacatgtatcaataatgtgaacaagagcatggagggaagcccaagccaaagaaagcaataagcactgcatgggcaaggagaatcaggaagggaagctcccccagcctgcagcagagtggtgcctaactagtgatttgtgaagatggctaaaaggaggaggtgtgctgtgagagggcagcgcaggcacaggcacttgcaccatcaatgacatcttgaccctacagagccaaatggagatgggcgtccagctcccaggaggtggatttgtggatctaagcctcatgttacttctcagctgaattgaaagaaacagctacaaatccccaaagtacaaagagatgctaagcaagaacaggtgttcttgtggccagagcatcaaaagcaacacgtacctgtcatgtcccacttgaggagaaactagttctacttgtatgcaagtatgtgagtgataaatacataaatggttatgaatgctaacaaagtgctgtttattggaatttggagtctcagaaattggctcttcactcaaagatttcaaaataatgcactcctgcttttagttagcattaactatattttttatcagttggaaaatagctacctatgtaatagagaacatcgaactgaagaaaaccagagaagacttcataaaggaaagttctctcccattttctccctcctgctaaactgctccaacccctttctcactttcttccaaaatacaaatgtcctcctaaacagccctcttttctgagttgcagatcaaatgtctggaaatcctccatctgcaggtgacaatgttgaaagatctagcaaggccttctcctcctgcaacattccatatatgaactaatgatatcaccacttctctgctgccatttctaaaccacaaggcttgcccagggcctctcaaaacccactgtccatgactgtatctccacttattttcccttagctaaaaatgtgttctcccctgaactgctttccctgtgccccttgtatcaaggttgctcattcttttcatcctcatatatttaagggtaaggagttcatatcagtgtcttcttcattccccatagtaccttctcaatcattcccaccccaatgtgtttgtaaaaatctatacctctctgaatctggtcccatttttctgtacaacttattgtggacatctgtgagttaccaacacagcattcattctatcatgtgcccttgttaactatacttcaatttttttcaacagtgacccatccccctacttatgccctaaagtcaactttttgataaactgactttagttctacctctagaattagtgtatgcatttacctggccacattgatggccttaggcataatcttatcagagtgaagctcaaaacttttgttcagtggttgcaggaaatggacactttttcttccacgagaggcaaactaggaagaatggattcaccattgctgctgatacctgtcttgcaaccaggaggaaaatcagcctaaagaaaaaactaacatataaaggaaagaagaaccaaagaaacaggaaaaaagaaaatgtagaaccaagacctgattgaatagttcctgaaacaactttacttgtggacttttctgtttgtctttaagtcacttgagatgggttttctgtactttcattgactttgtcatcactagaaactgttccttttcaaattcctactttaaaaatcctatcctcagacatcagcctcctgtcctttcagtttgttcacttacacatactacagtactaattagaatgtcatatctgttgaccatttttactatccacctactccttcctattttcatatataagttttgttcaccagtgggccaacccatgtagctcagtgtcttacatttagtaggcaattaataaattgtgttgattcattggttaattgattgttctctttgcctttctctctcaccccttcccaagtatgcttcacctagtgattattcttttaaattttttccataattatttttctgtaacacaatatatccttattactgtcccactggaaatcttcaataacactcattttgtccatagctggacctcagatgtggtccacactatgttcctgatgttgttgctttctaaaggttatcatcttccaattgagattgaggatggacaaacccttcctgaaccaaattcagtgctggaagccaccttaaaatgtcaacttcaaatatggtctaaaataatgtacttttaataaataaatataactctccatcatcacaaacctcagaaaagccatgcaatgatctctcctgcagtatctaattttgtaagaattccattctagacattatgctttaatggaacactggcaaaataaaagttatccaaagagtaaccaggatggtgaaaagcccagaaaccatgtgtcaaggggaaaacagggtttctttgcagagagagggtgtggggaccataacatttatgttctgatatttgaaggactgtcaagtggaagaacaaaagttgcaattctcttctgctccagacatcagaaaaagattaaatttaatcttatatggagttatatcttagctcaatatgaaatgtaacattaaaataatgtttctatccaggtatccagctataaaaggggcttacataaaagcagagttttataaagtatcaatcaagttagtctagtttgtgctgtagcaacaaagaacccccaaatctcaatggtatatcaaaaaaagtttgtttcttatttatactactttatttgtccagcacaggtcacaaaagatcctacgcattgtagccttcaaagactcaagatgacagaagatccaccatcctatgacactgccatctaaacacaagtctccagcggccactgtggcaaggaaacagagcttgaatcataaatcagctcttaaatgcttctgcctggaagtgattcacatcacttcacttaaatttcattggccaaagcagtccatggccatgtataatttcaaggagatgagacagctgtaaaaggaaggatgtcagaagcttcagttagcacttggaacatctaccataactttcagtaggatttaagcagaattcaaattctcattaggaatatcatagaaaaagttagattgctaagcctctttaaactctaggattctataattccaaacttatgtcagatagttcctttaatatcagggattttgcttcctagggtaaaatgaataactctggagcactgaaacttcccatatacaaaggactatgctcaatatttgaatttactgagctgagcttacaaagacttggcttggaagagctaaatattggcaggtcaacagccctaactctgtaagcttgttatggtccatttttttcaaacattgcttcaaatatttacatttgacttttacataaaagttgctgattttcagtagaggctgagatgaacgacagttgataactgttcctcatgttctatagaatttatgtgtaaggtttccagctatttttctatcttccttggtaagactgtagtgtagctaaacaggtggacttaaatgtcagctgtattctagtggcttaataatgcctttgaatacgtaatagccaatgcttacaggttatgttattttatattacagtctcctgtttaattttactgcagatacgtcttaaattgagagcaattactcccttcatttttgccattttaaacctgctgtgtactcattttttttaaattatgggccaaaaaaggacagctatacattttcagtgtcatggatctagagttatagctctagaggggccacagagatcacctagtttgcccctttgttttacatacaaaaaatttaagaacagttaacatttgttgagagtgtaccatgttctgggcactggcctactgttttctcatgtattaactcaactgatcttctcaatagcccaagaaaataaatactgtcatcatctccatttcacagatgaataaacttacctaagattgggaaacatttcccccttattagacaggtcaatattttaaaaaaaaaaatggcatagcctggtgctggggagaacacgaacaggcacatggcctcatttactgttcagcattttgtgacatttagctcaaactttttgatattgaatcttcctccatttctccacagttcttacatatcaatttggacaaaggtgacaagataatagcaaattccaagaaaaactattacatagttcaaataatcacacaattacatattagacagaaagtaaaggctagagaaagtctgcagcactacctaatctgagaaaatgattgggaaggaatgttaaaattattaaccattgaggcttgggccctaggctcccttactgggaagtttctggaatagtttctagagttatgtctgaaatagttttccaattctgattgaaacctttaagctaataatgcttacctatgaatgaagagatttgggtgacttttacatttttctttgtacttttcaatattgtttaattttccattgcagtgacaatacattttataaaatcatcgagaagatttaaacaaatgcaatgagtttattgaatgagctgaactcaggaagatagcaaaaagcaactttgttctttctcaccctgtacctgcatacctgttctttgggtttcatttaacaagctattctacaacctaagagataggcactaccctcccactcctgaggtctaccacttttagaactgtctactattgtcaacactacctgcgacccagtcttcggcatcccctcctcaaactcatccccctaaagttccagtctctgtcctgctcagacacctgtgtcagggctctctccagtgattctgaattgagtgcccttgggcacccctggtaagagcctctgtctactcaaccacacccagagctaccattcgctgtatgaagctggaaaagttcacaccccttagctctggtgctgaagtggacacgggtagagcacaggaaaatgtgctccctacatcccaaatgaaagccctgaactaatagaaacaaatgatgaggaggctctgtatcactgaagtatggacacattgtgggttaaaggctttggcagactgaactggagacataaccttcattcatcacacaatttctatagaaaaatgtgtcgagttcaaaacaactgacctacaaatgatccttaggaacataatttgtctggaaactgggggctgcttttataaccatctccagcctgtcagatccaatagattagagtcaagacagcacctttgatttacagtcttggccctgttgctgaagcacttcctaattcacactctctattcttaaaatgagaggcataatatgtctgctccaactacaaggttgttgagataataagcatggctatttctgagaaaatatcttacaaaattgacaatataagtgtttactattatttcatgtggtgcattacagaattcacagtacaggtaattggttatagggaagtcgtttctgagattaataagactgccgcaaaagtatcacaatatgctcctgttttttccccattcctgatttctttccttagcaaaaaatgttcctttgtctttcttaacctatgcatttttaggttattggcttttagaatattggcattactgaaaccctgtctaactttaggagcgctaattgagtatataataacacacatgtaaatcaacaaattttagaaagccttagaatctgcaaaaagcatgaaacataatttatcctatgctaagtacagtaactaggtaatgccagtgttaaaaaaaaaagtataaaacttgaaaataaggataaaagggtagagcaagcccttttgatgtctactggtatattatttcaatagtccacttcatgacaatttatctgattactcatgtttgactttgctatttcctatttgattagagactagacactatggaattatatgttaaattgtagatttttgttaagtaaaaaagataaccttaaagatggctgttctgttgtcccgtgggccactaaccaatgttgtatccaacccagctatcctattctaatatccttttaatgtctttcctgctgtactatatatatcattgttccttaaatgctcttggaaccagtttcatcctcatattggtatgtatgtatatgtatacatatatacacatatatgtatatatgtatacattatctgtaaacataataaagtgctttgaagaaattttaaaaataggaaagtgggtggtgccaaggaagctgagggaagaaaatgtttgagaagggaatgctcagaagaggctgcactgccataagttgaagggacttagcagtaaggaataggtcagtaaccttggagagagcagcattcatggggtggtgaaggcagaaaccgcatcattaagagcaaggggaagagggccagaacgtacacaccactttagggaagttggaatgtggggagagcagtgcaatgagatggtgccagatagataagagatccaaggagaggtatatattttgtgtgttttctgggttttttgatgttgtttgttttaatgggtgagaccagagtatatttaaatgcagatgggaagaacagtttgaagatcaagtaagagggatggaggtgggggtgaataattaaaagaaaaaagattcctgaggaggcaagaggggatagaatcccaagaacagatatttcagggtgggggcggggctggcaacagacagcatgttggctggctgaagttacggtgggaggtggtgggagttgtaagtctgaggagcttgtgaaatgtttcagatggaagctgtgggaaatagaagaaagctaaaaaacacacatgaattgcaaaatagcattgaggaccccagtacaagttgaatgcaatgacatcatagtggcaccaatatgattatatgaggtttttttttctccagccatgctcaagacttcagcttagccaaggaaatagcaggcacggtaggtattttctggctggttatgagtggaatataatgagagaaggtaaataggacacttatagggaggtaactgaagcaatggactaagcacttgtccaaacatttttgttctcatgctctcaaaagattttggaaaactatttctcacatattttgaaatcaaaatctaaaaatttttaacacataaagtgaaatagtttcaaaggatgtatttatggcttatattatatatgtacattaaatatatttttatccaagtcttggagttgtagatttagctcattctatttatagaacacgtctttcagataatcaggccacattgtgaaactaatcagccaaatcagggttacttttcatcagaaccagtacaattttattttaaaattcatacagtcatgcatctgtggaatacttctgtattctaagataggttaattgatttttaaatggatggttgattgttgggtagatagctggtggatagatgaataaaacaagacatggatggatagacaaattcttatcttgagtttgtctcctggataaaacaagatcccctcaaatatttctctctgaagtttttttttattttactttcaagagactttccctcaagaaagtggtattctagatttgtccctctttttgatgccccaagtgtttttacaccctggagcaatgcatcaaaatacaacttaggatgggggaagtacacttttcttttgtaaagtggagaagggcaatgtgaaaggtgaaaaaggaaagactaattggtagacatcagagtttgtatgcaggtcagcttgaagaatgaatatgaggaagttgagatttagaaatttctacactacagctttctaagcttttttgattatcccacaggtacctaaaacttaacatgcctaaaattgaacttacatatctacctcatcctagtcctccttcctcagtgagtggcaccatttctattcattaagacaagacagaaacctggcagtcaccctgaacttcttgttctctcatgcccttcatatccaactaaacaccaagatctggacattttttctcataatgatctcctgagtcagcccacatccctctatccccatggctatctctctgctgcagggtatggttgcctctcactcagctgccaaaatctgcctgtctctagtcttgagtcctctccacctgctctccatactacaaccagagaaagtattctaaaacatgtctgactaaatagctccatttttaaaaagttatcaatgacttcctataaccctaggccttattattcacttactagattactatttcaatcaagctctaaggacaaatcctaaactcattggcatggctttcaaggcccttctgaacttggcctctgctcatcatggcagcttccgctctccccactccatactctgcttatgaagtgttttcatcccaagtctcaccaggctctcctgcctcaaacactctttctgcctccttcttctagctccctcctatttagcattaaggtttcagctgagatgtaatttcctctagaaagcttttcctaatccctcaagtttgggtttgatccttatcttacatacttctgtgacgcattgtttgtagtccattatagcatttactctacattgagttttaactgtttacatgtctgaatacccaagagcagagggacatatgtgtgtgtctattcacttttgtattgtcagtgtctagggtactagccactgcctggtgcagagtaggtatccaataaacacgtacttaccgaataaatacgtgaagctaccaaaattttgcccccaaaataaatcacattccttctatgagtggcttataaacctgtttagtgaccaaatataaagttttcatcaagttcatatgaaattgttggcaaaaaataatccataagcttgatggggaaaaaattccatgccccatctctctaacaatgatatcaaaaactacttccttatacatagcaaaataacttagctgagaactgagtcaaaaggaactgaaattttcattattttattaattcattcaatgatcaatggtcacttagctctgccttcatgaagcagtgttgctctagtctagtctaatgcttgccccatgaagcccactgaaccctggagaaaagctggcccatctcttcagctttccaaattttattatatagaactaggagcagctgcttttatccaagtaggaataatttttaaatagcatttttccttgtatgtcagaaaacccaagctgaaaatattacatttcttaaaacttctatgctcctgatctttttcttcttttctgttgtgccagaggcatgaactttatgcccccagcaccagttaagaagatgatttattaaacagacttaaatgaaagatggcttggtgtggatacacttagattcacagaccgtgccttggggcagttttagtgccaactttctaactaattcagaaatgaaaaacttctcattatttcaggataaatgtctaaacctaccagctcttgtctgaatgacataaaagtatcagcactaaaaatggagattttgttgttcacatgtcatctagactctcaaccctacaatgtttaacatatgagccagttacaaattaccaactaatggtatcttttgggcacttccaggtaaagcctcccagtgtccattgtatcaaactctttccctttcatacagggttacctgtacagtagtatcactcagaagttatgctggaggaattgctttcaattttttcattaggttcataaaatctactcagaaaatagatttaaaacacaaatgttaaaatccatgcaaaaacacaaatattttgatttgatttatgcaaagccctaagcctgtgctgtgcacagagaagagagcaatggcatgactacttgtctgtttactctcagaatgtgcatatatgcatttcatttccttgatttgaccctaattcaaggggccagtctgaagagtcagcaatgttaatttactagatctcaaaagtaagtattcatattactgcaaaaagcaagatgtcattttctcatcatttctgtgaatagaaaagctattttccaacaatagggatcccttataatagggaaatacttaactggtactgaactcagaaactgcagtgttctgcttggcttcattgattttatcaaaggacctctttatcctgagcaggtaaagctcaatgaattgaaatagtccagaaatacatgaatagctgtcctctgacagaaagtaagtttaaattgtaagaaaattactttatttccaaggattcccgagattcttgttcctgattatggtccaaaattccacacagatttgttcttgattcatttcagagtagtcagaaaaggtactgttctccttacatagagaaagaacatcctgtggtttcatctcagaactgtagctctcatatttgcaacagaaaaaagctggaccaacagcacactaatggctttttgtgaacccatcagaaagctaaagtcgaaggataatagtcttcctgaaatctagagagatgtggggtacctatgtaaaaattagagggctgtggtggacacaggaatcataaaatcagccagtccttttgctgaaatacatttctagtagtgccatgggtgatttgaaaatagtcttgttccttttcttcattcccttgcacactctgtctcctcttctccatggctttataaattacacacagaattaaggcttcccatttaggagaacatccatttctctctgacaacgtcatcaaagaagtgttcttcttccaagattttctcttgatgcagggaagtggcaaagttctagaagatcatcaagggctggaaatattgctgtggtcattccagagaaatgcaatctaaacaggtcaccaattctttccaactatggcagacatcacaaatcaaatgatactccttccagtagaatgaggacaacctcaaaatctttcttaacatagtacttctcagcctgcaaaactaaaactcttgtaaacaggggctcgaataagtaacctatcacaattgataaaccacaccatgttgttggcaacctgatatgtgcaaggcattaaacggagagctttgccctcaaagggttaagaacatctagaatgggggtctcctctttcgtcttgggagccccctccgtctgtctctgtagtggggagcttcttccttcagccttcttccttctttcttgcctattaaattctccgctcagatgtgactgggcgcagcggccaccgtaaggcgtaaggggtgccaagtgccggttccagtcccg

SEQ ID NO: 18802 - RNA, 14091 nt, Homo sapiens
  source 1..14091: mol_type = other RNA
tgatggataaaagactacatattgggtacagtgtactctgctagggtcatgggtacatcaaaatctcagaaatcaccactaaagaacttatccatgtaagcaaacaccacctgttccccaaaaactattgaaataaaaaataataacaataaatatctttaaaaatatgactctatttaaatgttgagataaaatgaggctctattttccacgaagaaattaataatgctaaaattaagaattccagtttctccaataaacaattatatatttaacaaaaagtagtttattaatcacctttgttattgctgatatttatcccattgatttagaatcactactgccttcctgagagctaaacatctctttaatcaaataacatttttattttttgcttattatttgaacatgtgccttaaaagcactgcctattttgtttctaataagatatttatttttacctattttttacattgcagatttgttccactgttgttgttgtttttgtttcaggtatagaatgccacatactacataaaatgattctttttgcttatgaataatgtcaccaatttttaaaataacttgcagaaaacaaaactatgactaggcgttttcagtaaaaatgctaacattttggcaactttgtgaaattgtttattcctcctgatggtgtatacaacagagaaatgtggagaaaatgttctactaagaactcaatgataatttgctctacctatcacattttttaaattccatgtggttgtctccattaacggatggttaaacagctccaatttgaagacaaaatctttgattttttaggaaacaaatttttggagtatcagataatcattagttttcttatgacttgcaaaaaatttaccttggttatagtggtagctagggtcagacagattaattatattaaggctagacagtactatttttgaaggtagtttctcttcccttttaatagtaatgaattatttaaacaggaatcatgtaactaacacttagcactgttctaagaactttccgtatattacctcaattaattatcatgtaaatccagcaagttaataacttttaaaactcctattttacagataaacaatttgtagcacaaagagataaacagcttgcccaaagtcacacagctaggaagggggatcccagaattaaaactcaagcattctgcacttaaaattactacacaatactggcccactagcttaccatgttccatggcagaatccaatcattttacccacggccattctttaataatggcttcgaacttcttactccatgacctttgctgcttattttctcatgcacaccacagaccacactggactcattccttccacaagaactctgccccttgaatagagaagagcttttaaaatcgtaagtcaggactcacatcttctctataatattctccctaagtgtagtaaaccattgaaatgttcaatattatatgcctattctaattacttggagtagttgtcaataatacagtattgagaaatatcttgagaaaaaaaactagccttactagataagtgcttgatcattagcaacttttgttctgaccacagaacaactcatagcaagctgtaagtttgttccccctgctactgaaaccaatgccaaagtatgaaatatgttaccttgctcctaaaagcaatgagacataaaatagttggcttaataataacattaaaaaattctatttaaaagcaagctatacttcattatccccatcttctgatttaatatattagataggcatttatctataaacttacttgatcaaatatttgagtgaccatgatacccaaggcactgtgctggtactgcagagaatacagggccgaggaaatgatcttgtactcaagtatagaaagcagaacactttttttttttgtgaagatatgatggttacagtagtatgactgttagatgcatgaactcagataggacagacatacaatcaaccacataaggcagaaactgataaatactaaaagaaaaaaaaacaaatattaggcagaaatgtggaatattattgaatcatatattcaaatataataattaaaataaatctaacataagaataagaatgtgagaggatgcaatgtgggaaactacttaaagcttgaggagataacatgtatcaataatgtgaacaagagcatggagggaagcccaagccaaagaaagcaataagcactgcatgggcaaggagaatcaggaagggaagctcccccagcctgcagcagagtggtgcctaactagtgatttgtgaagatggctaaaaggaggaggtgtgctgtgagagggcagcgcaggcacaggcacttgcaccatcaatgacatcttgaccctacagagccaaatggagatgggcgtccagctcccaggaggtggatttgtggatctaagcctcatgttacttctcagctgaattgaaagaaacagctacaaatccccaaagtacaaagagatgctaagcaagaacaggtgttcttgtggccagagcatcaaaagcaacacgtacctgtcatgtcccacttgaggagaaactagttctacttgtatgcaagtatgtgagtgataaatacataaatggttatgaatgctaacaaagtgctgtttattggaatttggagtctcagaaattggctcttcactcaaagatttcaaaataatgcactcctgcttttagttagcattaactatattttttatcagttggaaaatagctacctatgtaatagagaacatcgaactgaagaaaaccagagaagacttcataaaggaaagttctctcccattttctccctcctgctaaactgctccaacccctttctcactttcttccaaaatacaaatgtcctcctaaacagccctcttttctgagttgcagatcaaatgtctggaaatcctccatctgcaggtgacaatgttgaaagatctagcaaggccttctcctcctgcaacattccatatatgaactaatgatatcaccacttctctgctgccatttctaaaccacaaggcttgcccagggcctctcaaaacccactgtccatgactgtatctccacttattttcccttagctaaaaatgtgttctcccctgaactgctttccctgtgccccttgtatcaaggttgctcattcttttcatcctcatatatttaagggtaaggagttcatatcagtgtcttcttcattccccatagtaccttctcaatcattcccaccccaatgtgtttgtaaaaatctatacctctctgaatctggtcccatttttctgtacaacttattgtggacatctgtgagttaccaacacagcattcattctatcatgtgcccttgttaactatacttcaatttttttcaacagtgacccatccccctacttatgccctaaagtcaactttttgataaactgactttagttctacctctagaattagtgtatgcatttacctggccacattgatggccttaggcataatcttatcagagtgaagctcaaaacttttgttcagtggttgcaggaaatggacactttttcttccacgagaggcaaactaggaagaatggattcaccattgctgctgatacctgtcttgcaaccaggaggaaaatcagcctaaagaaaaaactaacatataaaggaaagaagaaccaaagaaacaggaaaaaagaaaatgtagaaccaagacctgattgaatagttcctgaaacaactttacttgtggacttttctgtttgtctttaagtcacttgagatgggttttctgtactttcattgactttgtcatcactagaaactgttccttttcaaattcctactttaaaaatcctatcctcagacatcagcctcctgtcctttcagtttgttcacttacacatactacagtactaattagaatgtcatatctgttgaccatttttactatccacctactccttcctattttcatatataagttttgttcaccagtgggccaacccatgtagctcagtgtcttacatttagtaggcaattaataaattgtgttgattcattggttaattgattgttctctttgcctttctctctcaccccttcccaagtatgcttcacctagtgattattcttttaaattttttccataattatttttctgtaacacaatatatccttattactgtcccactggaaatcttcaataacactcattttgtccatagctggacctcagatgtggtccacactatgttcctgatgttgttgctttctaaaggttatcatcttccaattgagattgaggatggacaaacccttcctgaaccaaattcagtgctggaagccaccttaaaatgtcaacttcaaatatggtctaaaataatgtacttttaataaataaatataactctccatcatcacaaacctcagaaaagccatgcaatgatctctcctgcagtatctaattttgtaagaattccattctagacattatgctttaatggaacactggcaaaataaaagttatccaaagagtaaccaggatggtgaaaagcccagaaaccatgtgtcaaggggaaaacagggtttctttgcagagagagggtgtggggaccataacatttatgttctgatatttgaaggactgtcaagtggaagaacaaaagttgcaattctcttctgctccagacatcagaaaaagattaaatttaatcttatatggagttatatcttagctcaatatgaaatgtaacattaaaataatgtttctatccaggtatccagctataaaaggggcttacataaaagcagagttttataaagtatcaatcaagttagtctagtttgtgctgtagcaacaaagaacccccaaatctcaatggtatatcaaaaaaagtttgtttcttatttatactactttatttgtccagcacaggtcacaaaagatcctacgcattgtagccttcaaagactcaagatgacagaagatccaccatcctatgacactgccatctaaacacaagtctccagcggccactgtggcaaggaaacagagcttgaatcataaatcagctcttaaatgcttctgcctggaagtgattcacatcacttcacttaaatttcattggccaaagcagtccatggccatgtataatttcaaggagatgagacagctgtaaaaggaaggatgtcagaagcttcagttagcacttggaacatctaccataactttcagtaggatttaagcagaattcaaattctcattaggaatatcatagaaaaagttagattgctaagcctctttaaactctaggattctataattccaaacttatgtcagatagttcctttaatatcagggattttgcttcctagggtaaaatgaataactctggagcactgaaacttcccatatacaaaggactatgctcaatatttgaatttactgagctgagcttacaaagacttggcttggaagagctaaatattggcaggtcaacagccctaactctgtaagcttgttatggtccatttttttcaaacattgcttcaaatatttacatttgacttttacataaaagttgctgattttcagtagaggctgagatgaacgacagttgataactgttcctcatgttctatagaatttatgtgtaaggtttccagctatttttctatcttccttggtaagactgtagtgtagctaaacaggtggacttaaatgtcagctgtattctagtggcttaataatgcctttgaatacgtaatagccaatgcttacaggttatgttattttatattacagtctcctgtttaattttactgcagatacgtcttaaattgagagcaattactcccttcatttttgccattttaaacctgctgtgtactcattttttttaaattatgggccaaaaaaggacagctatacattttcagtgtcatggatctagagttatagctctagaggggccacagagatcacctagtttgcccctttgttttacatacaaaaaatttaagaacagttaacatttgttgagagtgtaccatgttctgggcactggcctactgttttctcatgtattaactcaactgatcttctcaatagcccaagaaaataaatactgtcatcatctccatttcacagatgaataaacttacctaagattgggaaacatttcccccttattagacaggtcaatattttaaaaaaaaaaatggcatagcctggtgctggggagaacacgaacaggcacatggcctcatttactgttcagcattttgtgacatttagctcaaactttttgatattgaatcttcctccatttctccacagttcttacatatcaatttggacaaaggtgacaagataatagcaaattccaagaaaaactattacatagttcaaataatcacacaattacatattagacagaaagtaaaggctagagaaagtctgcagcactacctaatctgagaaaatgattgggaaggaatgttaaaattattaaccattgaggcttgggccctaggctcccttactgggaagtttctggaatagtttctagagttatgtctgaaatagttttccaattctgattgaaacctttaagctaataatgcttacctatgaatgaagagatttgggtgacttttacatttttctttgtacttttcaatattgtttaattttccattgcagtgacaatacattttataaaatcatcgagaagatttaaacaaatgcaatgagtttattgaatgagctgaactcaggaagatagcaaaaagcaactttgttctttctcaccctgtacctgcatacctgttctttgggtttcatttaacaagctattctacaacctaagagataggcactaccctcccactcctgaggtctaccacttttagaactgtctactattgtcaacactacctgcgacccagtcttcggcatcccctcctcaaactcatccccctaaagttccagtctctgtcctgctcagacacctgtgtcagggctctctccagtgattctgaattgagtgcccttgggcacccctggtaagagcctctgtctactcaaccacacccagagctaccattcgctgtatgaagctggaaaagttcacaccccttagctctggtgctgaagtggacacgggtagagcacaggaaaatgtgctccctacatcccaaatgaaagccctgaactaatagaaacaaatgatgaggaggctctgtatcactgaagtatggacacattgtgggttaaaggctttggcagactgaactggagacataaccttcattcatcacacaatttctatagaaaaatgtgtcgagttcaaaacaactgacctacaaatgatccttaggaacataatttgtctggaaactgggggctgcttttataaccatctccagcctgtcagatccaatagattagagtcaagacagcacctttgatttacagtcttggccctgttgctgaagcacttcctaattcacactctctattcttaaaatgagaggcataatatgtctgctccaactacaaggttgttgagataataagcatggctatttctgagaaaatatcttacaaaattgacaatataagtgtttactattatttcatgtggtgcattacagaattcacagtacaggtaattggttatagggaagtcgtttctgagattaataagactgccgcaaaagtatcacaatatgctcctgttttttccccattcctgatttctttccttagcaaaaaatgttcctttgtctttcttaacctatgcatttttaggttattggcttttagaatattggcattactgaaaccctgtctaactttaggagcgctaattgagtatataataacacacatgtaaatcaacaaattttagaaagccttagaatctgcaaaaagcatgaaacataatttatcctatgctaagtacagtaactaggtaatgccagtgttaaaaaaaaaagtataaaacttgaaaataaggataaaagggtagagcaagcccttttgatgtctactggtatattatttcaatagtccacttcatgacaatttatctgattactcatgtttgactttgctatttcctatttgattagagactagacactatggaattatatgttaaattgtagatttttgttaagtaaaaaagataaccttaaagatggctgttctgttgtcccgtgggccactaaccaatgttgtatccaacccagctatcctattctaatatccttttaatgtctttcctgctgtactatatatatcattgttccttaaatgctcttggaaccagtttcatcctcatattggtatgtatgtatatgtatacatatatacacatatatgtatatatgtatacattatctgtaaacataataaagtgctttgaagaaattttaaaaataggaaagtgggtggtgccaaggaagctgagggaagaaaatgtttgagaagggaatgctcagaagaggctgcactgccataagttgaagggacttagcagtaaggaataggtcagtaaccttggagagagcagcattcatggggtggtgaaggcagaaaccgcatcattaagagcaaggggaagagggccagaacgtacacaccactttagggaagttggaatgtggggagagcagtgcaatgagatggtgccagatagataagagatccaaggagaggtatatattttgtgtgttttctgggttttttgatgttgtttgttttaatgggtgagaccagagtatatttaaatgcagatgggaagaacagtttgaagatcaagtaagagggatggaggtgggggtgaataattaaaagaaaaaagattcctgaggaggcaagaggggatagaatcccaagaacagatatttcagggtgggggcggggctggcaacagacagcatgttggctggctgaagttacggtgggaggtggtgggagttgtaagtctgaggagcttgtgaaatgtttcagatggaagctgtgggaaatagaagaaagctaaaaaacacacatgaattgcaaaatagcattgaggaccccagtacaagttgaatgcaatgacatcatagtggcaccaatatgattatatgaggtttttttttctccagccatgctcaagacttcagcttagccaaggaaatagcaggcacggtaggtattttctggctggttatgagtggaatataatgagagaaggtaaataggacacttatagggaggtaactgaagcaatggactaagcacttgtccaaacatttttgttctcatgctctcaaaagattttggaaaactatttctcacatattttgaaatcaaaatctaaaaatttttaacacataaagtgaaatagtttcaaaggatgtatttatggcttatattatatatgtacattaaatatatttttatccaagtcttggagttgtagatttagctcattctatttatagaacacgtctttcagataatcaggccacattgtgaaactaatcagccaaatcagggttacttttcatcagaaccagtacaattttattttaaaattcatacagtcatgcatctgtggaatacttctgtattctaagataggttaattgatttttaaatggatggttgattgttgggtagatagctggtggatagatgaataaaacaagacatggatggatagacaaattcttatcttgagtttgtctcctggataaaacaagatcccctcaaatatttctctctgaagtttttttttattttactttcaagagactttccctcaagaaagtggtattctagatttgtccctctttttgatgccccaagtgtttttacaccctggagcaatgcatcaaaatacaacttaggatgggggaagtacacttttcttttgtaaagtggagaagggcaatgtgaaaggtgaaaaaggaaagactaattggtagacatcagagtttgtatgcaggtcagcttgaagaatgaatatgaggaagttgagatttagaaatttctacactacagctttctaagcttttttgattatcccacaggtacctaaaacttaacatgcctaaaattgaacttacatatctacctcatcctagtcctccttcctcagtgagtggcaccatttctattcattaagacaagacagaaacctggcagtcaccctgaacttcttgttctctcatgcccttcatatccaactaaacaccaagatctggacattttttctcataatgatctcctgagtcagcccacatccctctatccccatggctatctctctgctgcagggtatggttgcctctcactcagctgccaaaatctgcctgtctctagtcttgagtcctctccacctgctctccatactacaaccagagaaagtattctaaaacatgtctgactaaatagctccatttttaaaaagttatcaatgacttcctataaccctaggccttattattcacttactagattactatttcaatcaagctctaaggacaaatcctaaactcattggcatggctttcaaggcccttctgaacttggcctctgctcatcatggcagcttccgctctccccactccatactctgcttatgaagtgttttcatcccaagtctcaccaggctctcctgcctcaaacactctttctgcctccttcttctagctccctcctatttagcattaaggtttcagctgagatgtaatttcctctagaaagcttttcctaatccctcaagtttgggtttgatccttatcttacatacttctgtgacgcattgtttgtagtccattatagcatttactctacattgagttttaactgtttacatgtctgaatacccaagagcagagggacatatgtgtgtgtctattcacttttgtattgtcagtgtctagggtactagccactgcctggtgcagagtaggtatccaataaacacgtacttaccgaataaatacgtgaagctaccaaaattttgcccccaaaataaatcacattccttctatgagtggcttataaacctgtttagtgaccaaatataaagttttcatcaagttcatatgaaattgttggcaaaaaataatccataagcttgatggggaaaaaattccatgccccatctctctaacaatgatatcaaaaactacttccttatacatagcaaaataacttagctgagaactgagtcaaaaggaactgaaattttcattattttattaattcattcaatgatcaatggtcacttagctctgccttcatgaagcagtgttgctctagtctagtctaatgcttgccccatgaagcccactgaaccctggagaaaagctggcccatctcttcagctttccaaattttattatatagaactaggagcagctgcttttatccaagtaggaataatttttaaatagcatttttccttgtatgtcagaaaacccaagctgaaaatattacatttcttaaaacttctatgctcctgatctttttcttcttttctgttgtgccagaggcatgaactttatgcccccagcaccagttaagaagatgatttattaaacagacttaaatgaaagatggcttggtgtggatacacttagattcacagaccgtgccttggggcagttttagtgccaactttctaactaattcagaaatgaaaaacttctcattatttcaggataaatgtctaaacctaccagctcttgtctgaatgacataaaagtatcagcactaaaaatggagattttgttgttcacatgtcatctagactctcaaccctacaatgtttaacatatgagccagttacaaattaccaactaatggtatcttttgggcacttccaggtaaagcctcccagtgtccattgtatcaaactctttccctttcatacagggttacctgtacagtagtatcactcagaagttatgctggaggaattgctttcaattttttcattaggttcataaaatctactcagaaaatagatttaaaacacaaatgttaaaatccatgcaaaaacacaaatattttgatttgatttatgcaaagccctaagcctgtgctgtgcacagagaagagagcaatggcatgactacttgtctgtttactctcagaatgtgcatatatgcatttcatttccttgatttgaccctaattcaaggggccagtctgaagagtcagcaatgttaatttactagatctcaaaagtaagtattcatattactgcaaaaagcaagatgtcattttctcatcatttctgtgaatagaaaagctattttccaacaatagggatcccttataatagggaaatacttaactggtactgaactcagaaactgcagtgttctgcttggcttcattgattttatcaaaggacctctttatcctgagcaggtaaagctcaatgaattgaaatagtccagaaatacatgaatagctgtcctctgacagaaagtaagtttaaattgtaagaaaattactttatttccaaggattcccgagattcttgttcctgattatggtccaaaattccacacagatttgttcttgattcatttcagagtagtcagaaaaggtactgttctccttacatagagaaagaacatcctgtggtttcatctcagaactgtagctctcatatttgcaacagaaaaaagctggaccaacagcacactaatggctttttgtgaacccatcagaaagctaaagtcgaaggataatagtcttcctgaaatctagagagatgtggggtacctatgtaaaaattagagggctgtggtggacacaggaatcataaaatcagccagtccttttgctgaaatacatttctagtagtgccatgggtgatttgaaaatagtcttgttccttttcttcattcccttgcacactctgtctcctcttctccatggctttataaattacacacagaattaaggcttcccatttaggagaacatccatttctctctgacaacgtcatcaaagaagtgttcttcttccaagattttctcttgatgcagggaagtggcaaagttctagaagatcatcaagggctggaaatattgctgtggtcattccagagaaatgcaatctcaagctaattgaagagcccttgggccttaagtgaacatcagtggaagcctggcagcactcctcataggccagtgatggtggtgtccacagggttaggatcctctgcctgtggaaagtggagggaagagcgggaaggcctgcatctcatgatttgagtgccagctcagcagcagtacaacagaacaccaggtagatgtctaaggttttttactccagtacatggctcatggatgacacctccggacccacccggggtctgggggaacttgccgccctgaaggaaaggacacaagtctgtcccactttgccacctgctgactgtaccgccctagagccttgagcaaacataggtagcacccaagtagtggttactgcaggccttcggcaagacttcatgctgtgctgacttcaggtctgacccagtgcagtcccagtggtggtcacagagctgcttgtgtcacccccatccccagccacaggtagttcatcgcagagacagaaactacttttgtttgggagaaaataaaggaagagaacaagagtatctgcctggtaatctagagaaatgtcctggatcttaaccaagaccagcaaagtagtacctatacaaatctacaagaaccacagcattagtggccttggggtgccccctaatggagatacagcttacatcacaacacccaagtcattctgaatacctgtaaagccttcccaagcaggacaagcacaaataagcccagactgcaaggactataagtaaacacctaactcttcaatgcctgacgaacatctacaatcatcaccaccacccatggaaaacatgacctcagcaaaccaactaaataaggtgccagacatcaatcctggagaaacacaaatatgaaacctttcagagaaaaaattcaaaatagctgtgttga

SEQ ID NO: 18803 - RNA, 14127 nt, Homo sapiens
  source 1..14127: mol_type = other RNA
tgatggataaaagactacatattgggtacagtgtactctgctagggtcatgggtacatcaaaatctcagaaatcaccactaaagaacttatccatgtaagcaaacaccacctgttccccaaaaactattgaaataaaaaataataacaataaatatctttaaaaatatgactctatttaaatgttgagataaaatgaggctctattttccacgaagaaattaataatgctaaaattaagaattccagtttctccaataaacaattatatatttaacaaaaagtagtttattaatcacctttgttattgctgatatttatcccattgatttagaatcactactgccttcctgagagctaaacatctctttaatcaaataacatttttattttttgcttattatttgaacatgtgccttaaaagcactgcctattttgtttctaataagatatttatttttacctattttttacattgcagatttgttccactgttgttgttgtttttgtttcaggtatagaatgccacatactacataaaatgattctttttgcttatgaataatgtcaccaatttttaaaataacttgcagaaaacaaaactatgactaggcgttttcagtaaaaatgctaacattttggcaactttgtgaaattgtttattcctcctgatggtgtatacaacagagaaatgtggagaaaatgttctactaagaactcaatgataatttgctctacctatcacattttttaaattccatgtggttgtctccattaacggatggttaaacagctccaatttgaagacaaaatctttgattttttaggaaacaaatttttggagtatcagataatcattagttttcttatgacttgcaaaaaatttaccttggttatagtggtagctagggtcagacagattaattatattaaggctagacagtactatttttgaaggtagtttctcttcccttttaatagtaatgaattatttaaacaggaatcatgtaactaacacttagcactgttctaagaactttccgtatattacctcaattaattatcatgtaaatccagcaagttaataacttttaaaactcctattttacagataaacaatttgtagcacaaagagataaacagcttgcccaaagtcacacagctaggaagggggatcccagaattaaaactcaagcattctgcacttaaaattactacacaatactggcccactagcttaccatgttccatggcagaatccaatcattttacccacggccattctttaataatggcttcgaacttcttactccatgacctttgctgcttattttctcatgcacaccacagaccacactggactcattccttccacaagaactctgccccttgaatagagaagagcttttaaaatcgtaagtcaggactcacatcttctctataatattctccctaagtgtagtaaaccattgaaatgttcaatattatatgcctattctaattacttggagtagttgtcaataatacagtattgagaaatatcttgagaaaaaaaactagccttactagataagtgcttgatcattagcaacttttgttctgaccacagaacaactcatagcaagctgtaagtttgttccccctgctactgaaaccaatgccaaagtatgaaatatgttaccttgctcctaaaagcaatgagacataaaatagttggcttaataataacattaaaaaattctatttaaaagcaagctatacttcattatccccatcttctgatttaatatattagataggcatttatctataaacttacttgatcaaatatttgagtgaccatgatacccaaggcactgtgctggtactgcagagaatacagggccgaggaaatgatcttgtactcaagtatagaaagcagaacactttttttttttgtgaagatatgatggttacagtagtatgactgttagatgcatgaactcagataggacagacatacaatcaaccacataaggcagaaactgataaatactaaaagaaaaaaaaacaaatattaggcagaaatgtggaatattattgaatcatatattcaaatataataattaaaataaatctaacataagaataagaatgtgagaggatgcaatgtgggaaactacttaaagcttgaggagataacatgtatcaataatgtgaacaagagcatggagggaagcccaagccaaagaaagcaataagcactgcatgggcaaggagaatcaggaagggaagctcccccagcctgcagcagagtggtgcctaactagtgatttgtgaagatggctaaaaggaggaggtgtgctgtgagagggcagcgcaggcacaggcacttgcaccatcaatgacatcttgaccctacagagccaaatggagatgggcgtccagctcccaggaggtggatttgtggatctaagcctcatgttacttctcagctgaattgaaagaaacagctacaaatccccaaagtacaaagagatgctaagcaagaacaggtgttcttgtggccagagcatcaaaagcaacacgtacctgtcatgtcccacttgaggagaaactagttctacttgtatgcaagtatgtgagtgataaatacataaatggttatgaatgctaacaaagtgctgtttattggaatttggagtctcagaaattggctcttcactcaaagatttcaaaataatgcactcctgcttttagttagcattaactatattttttatcagttggaaaatagctacctatgtaatagagaacatcgaactgaagaaaaccagagaagacttcataaaggaaagttctctcccattttctccctcctgctaaactgctccaacccctttctcactttcttccaaaatacaaatgtcctcctaaacagccctcttttctgagttgcagatcaaatgtctggaaatcctccatctgcaggtgacaatgttgaaagatctagcaaggccttctcctcctgcaacattccatatatgaactaatgatatcaccacttctctgctgccatttctaaaccacaaggcttgcccagggcctctcaaaacccactgtccatgactgtatctccacttattttcccttagctaaaaatgtgttctcccctgaactgctttccctgtgccccttgtatcaaggttgctcattcttttcatcctcatatatttaagggtaaggagttcatatcagtgtcttcttcattccccatagtaccttctcaatcattcccaccccaatgtgtttgtaaaaatctatacctctctgaatctggtcccatttttctgtacaacttattgtggacatctgtgagttaccaacacagcattcattctatcatgtgcccttgttaactatacttcaatttttttcaacagtgacccatccccctacttatgccctaaagtcaactttttgataaactgactttagttctacctctagaattagtgtatgcatttacctggccacattgatggccttaggcataatcttatcagagtgaagctcaaaacttttgttcagtggttgcaggaaatggacactttttcttccacgagaggcaaactaggaagaatggattcaccattgctgctgatacctgtcttgcaaccaggaggaaaatcagcctaaagaaaaaactaacatataaaggaaagaagaaccaaagaaacaggaaaaaagaaaatgtagaaccaagacctgattgaatagttcctgaaacaactttacttgtggacttttctgtttgtctttaagtcacttgagatgggttttctgtactttcattgactttgtcatcactagaaactgttccttttcaaattcctactttaaaaatcctatcctcagacatcagcctcctgtcctttcagtttgttcacttacacatactacagtactaattagaatgtcatatctgttgaccatttttactatccacctactccttcctattttcatatataagttttgttcaccagtgggccaacccatgtagctcagtgtcttacatttagtaggcaattaataaattgtgttgattcattggttaattgattgttctctttgcctttctctctcaccccttcccaagtatgcttcacctagtgattattcttttaaattttttccataattatttttctgtaacacaatatatccttattactgtcccactggaaatcttcaataacactcattttgtccatagctggacctcagatgtggtccacactatgttcctgatgttgttgctttctaaaggttatcatcttccaattgagattgaggatggacaaacccttcctgaaccaaattcagtgctggaagccaccttaaaatgtcaacttcaaatatggtctaaaataatgtacttttaataaataaatataactctccatcatcacaaacctcagaaaagccatgcaatgatctctcctgcagtatctaattttgtaagaattccattctagacattatgctttaatggaacactggcaaaataaaagttatccaaagagtaaccaggatggtgaaaagcccagaaaccatgtgtcaaggggaaaacagggtttctttgcagagagagggtgtggggaccataacatttatgttctgatatttgaaggactgtcaagtggaagaacaaaagttgcaattctcttctgctccagacatcagaaaaagattaaatttaatcttatatggagttatatcttagctcaatatgaaatgtaacattaaaataatgtttctatccaggtatccagctataaaaggggcttacataaaagcagagttttataaagtatcaatcaagttagtctagtttgtgctgtagcaacaaagaacccccaaatctcaatggtatatcaaaaaaagtttgtttcttatttatactactttatttgtccagcacaggtcacaaaagatcctacgcattgtagccttcaaagactcaagatgacagaagatccaccatcctatgacactgccatctaaacacaagtctccagcggccactgtggcaaggaaacagagcttgaatcataaatcagctcttaaatgcttctgcctggaagtgattcacatcacttcacttaaatttcattggccaaagcagtccatggccatgtataatttcaaggagatgagacagctgtaaaaggaaggatgtcagaagcttcagttagcacttggaacatctaccataactttcagtaggatttaagcagaattcaaattctcattaggaatatcatagaaaaagttagattgctaagcctctttaaactctaggattctataattccaaacttatgtcagatagttcctttaatatcagggattttgcttcctagggtaaaatgaataactctggagcactgaaacttcccatatacaaaggactatgctcaatatttgaatttactgagctgagcttacaaagacttggcttggaagagctaaatattggcaggtcaacagccctaactctgtaagcttgttatggtccatttttttcaaacattgcttcaaatatttacatttgacttttacataaaagttgctgattttcagtagaggctgagatgaacgacagttgataactgttcctcatgttctatagaatttatgtgtaaggtttccagctatttttctatcttccttggtaagactgtagtgtagctaaacaggtggacttaaatgtcagctgtattctagtggcttaataatgcctttgaatacgtaatagccaatgcttacaggttatgttattttatattacagtctcctgtttaattttactgcagatacgtcttaaattgagagcaattactcccttcatttttgccattttaaacctgctgtgtactcattttttttaaattatgggccaaaaaaggacagctatacattttcagtgtcatggatctagagttatagctctagaggggccacagagatcacctagtttgcccctttgttttacatacaaaaaatttaagaacagttaacatttgttgagagtgtaccatgttctgggcactggcctactgttttctcatgtattaactcaactgatcttctcaatagcccaagaaaataaatactgtcatcatctccatttcacagatgaataaacttacctaagattgggaaacatttcccccttattagacaggtcaatattttaaaaaaaaaaatggcatagcctggtgctggggagaacacgaacaggcacatggcctcatttactgttcagcattttgtgacatttagctcaaactttttgatattgaatcttcctccatttctccacagttcttacatatcaatttggacaaaggtgacaagataatagcaaattccaagaaaaactattacatagttcaaataatcacacaattacatattagacagaaagtaaaggctagagaaagtctgcagcactacctaatctgagaaaatgattgggaaggaatgttaaaattattaaccattgaggcttgggccctaggctcccttactgggaagtttctggaatagtttctagagttatgtctgaaatagttttccaattctgattgaaacctttaagctaataatgcttacctatgaatgaagagatttgggtgacttttacatttttctttgtacttttcaatattgtttaattttccattgcagtgacaatacattttataaaatcatcgagaagatttaaacaaatgcaatgagtttattgaatgagctgaactcaggaagatagcaaaaagcaactttgttctttctcaccctgtacctgcatacctgttctttgggtttcatttaacaagctattctacaacctaagagataggcactaccctcccactcctgaggtctaccacttttagaactgtctactattgtcaacactacctgcgacccagtcttcggcatcccctcctcaaactcatccccctaaagttccagtctctgtcctgctcagacacctgtgtcagggctctctccagtgattctgaattgagtgcccttgggcacccctggtaagagcctctgtctactcaaccacacccagagctaccattcgctgtatgaagctggaaaagttcacaccccttagctctggtgctgaagtggacacgggtagagcacaggaaaatgtgctccctacatcccaaatgaaagccctgaactaatagaaacaaatgatgaggaggctctgtatcactgaagtatggacacattgtgggttaaaggctttggcagactgaactggagacataaccttcattcatcacacaatttctatagaaaaatgtgtcgagttcaaaacaactgacctacaaatgatccttaggaacataatttgtctggaaactgggggctgcttttataaccatctccagcctgtcagatccaatagattagagtcaagacagcacctttgatttacagtcttggccctgttgctgaagcacttcctaattcacactctctattcttaaaatgagaggcataatatgtctgctccaactacaaggttgttgagataataagcatggctatttctgagaaaatatcttacaaaattgacaatataagtgtttactattatttcatgtggtgcattacagaattcacagtacaggtaattggttatagggaagtcgtttctgagattaataagactgccgcaaaagtatcacaatatgctcctgttttttccccattcctgatttctttccttagcaaaaaatgttcctttgtctttcttaacctatgcatttttaggttattggcttttagaatattggcattactgaaaccctgtctaactttaggagcgctaattgagtatataataacacacatgtaaatcaacaaattttagaaagccttagaatctgcaaaaagcatgaaacataatttatcctatgctaagtacagtaactaggtaatgccagtgttaaaaaaaaaagtataaaacttgaaaataaggataaaagggtagagcaagcccttttgatgtctactggtatattatttcaatagtccacttcatgacaatttatctgattactcatgtttgactttgctatttcctatttgattagagactagacactatggaattatatgttaaattgtagatttttgttaagtaaaaaagataaccttaaagatggctgttctgttgtcccgtgggccactaaccaatgttgtatccaacccagctatcctattctaatatccttttaatgtctttcctgctgtactatatatatcattgttccttaaatgctcttggaaccagtttcatcctcatattggtatgtatgtatatgtatacatatatacacatatatgtatatatgtatacattatctgtaaacataataaagtgctttgaagaaattttaaaaataggaaagtgggtggtgccaaggaagctgagggaagaaaatgtttgagaagggaatgctcagaagaggctgcactgccataagttgaagggacttagcagtaaggaataggtcagtaaccttggagagagcagcattcatggggtggtgaaggcagaaaccgcatcattaagagcaaggggaagagggccagaacgtacacaccactttagggaagttggaatgtggggagagcagtgcaatgagatggtgccagatagataagagatccaaggagaggtatatattttgtgtgttttctgggttttttgatgttgtttgttttaatgggtgagaccagagtatatttaaatgcagatgggaagaacagtttgaagatcaagtaagagggatggaggtgggggtgaataattaaaagaaaaaagattcctgaggaggcaagaggggatagaatcccaagaacagatatttcagggtgggggcggggctggcaacagacagcatgttggctggctgaagttacggtgggaggtggtgggagttgtaagtctgaggagcttgtgaaatgtttcagatggaagctgtgggaaatagaagaaagctaaaaaacacacatgaattgcaaaatagcattgaggaccccagtacaagttgaatgcaatgacatcatagtggcaccaatatgattatatgaggtttttttttctccagccatgctcaagacttcagcttagccaaggaaatagcaggcacggtaggtattttctggctggttatgagtggaatataatgagagaaggtaaataggacacttatagggaggtaactgaagcaatggactaagcacttgtccaaacatttttgttctcatgctctcaaaagattttggaaaactatttctcacatattttgaaatcaaaatctaaaaatttttaacacataaagtgaaatagtttcaaaggatgtatttatggcttatattatatatgtacattaaatatatttttatccaagtcttggagttgtagatttagctcattctatttatagaacacgtctttcagataatcaggccacattgtgaaactaatcagccaaatcagggttacttttcatcagaaccagtacaattttattttaaaattcatacagtcatgcatctgtggaatacttctgtattctaagataggttaattgatttttaaatggatggttgattgttgggtagatagctggtggatagatgaataaaacaagacatggatggatagacaaattcttatcttgagtttgtctcctggataaaacaagatcccctcaaatatttctctctgaagtttttttttattttactttcaagagactttccctcaagaaagtggtattctagatttgtccctctttttgatgccccaagtgtttttacaccctggagcaatgcatcaaaatacaacttaggatgggggaagtacacttttcttttgtaaagtggagaagggcaatgtgaaaggtgaaaaaggaaagactaattggtagacatcagagtttgtatgcaggtcagcttgaagaatgaatatgaggaagttgagatttagaaatttctacactacagctttctaagcttttttgattatcccacaggtacctaaaacttaacatgcctaaaattgaacttacatatctacctcatcctagtcctccttcctcagtgagtggcaccatttctattcattaagacaagacagaaacctggcagtcaccctgaacttcttgttctctcatgcccttcatatccaactaaacaccaagatctggacattttttctcataatgatctcctgagtcagcccacatccctctatccccatggctatctctctgctgcagggtatggttgcctctcactcagctgccaaaatctgcctgtctctagtcttgagtcctctccacctgctctccatactacaaccagagaaagtattctaaaacatgtctgactaaatagctccatttttaaaaagttatcaatgacttcctataaccctaggccttattattcacttactagattactatttcaatcaagctctaaggacaaatcctaaactcattggcatggctttcaaggcccttctgaacttggcctctgctcatcatggcagcttccgctctccccactccatactctgcttatgaagtgttttcatcccaagtctcaccaggctctcctgcctcaaacactctttctgcctccttcttctagctccctcctatttagcattaaggtttcagctgagatgtaatttcctctagaaagcttttcctaatccctcaagtttgggtttgatccttatcttacatacttctgtgacgcattgtttgtagtccattatagcatttactctacattgagttttaactgtttacatgtctgaatacccaagagcagagggacatatgtgtgtgtctattcacttttgtattgtcagtgtctagggtactagccactgcctggtgcagagtaggtatccaataaacacgtacttaccgaataaatacgtgaagctaccaaaattttgcccccaaaataaatcacattccttctatgagtggcttataaacctgtttagtgaccaaatataaagttttcatcaagttcatatgaaattgttggcaaaaaataatccataagcttgatggggaaaaaattccatgccccatctctctaacaatgatatcaaaaactacttccttatacatagcaaaataacttagctgagaactgagtcaaaaggaactgaaattttcattattttattaattcattcaatgatcaatggtcacttagctctgccttcatgaagcagtgttgctctagtctagtctaatgcttgccccatgaagcccactgaaccctggagaaaagctggcccatctcttcagctttccaaattttattatatagaactaggagcagctgcttttatccaagtaggaataatttttaaatagcatttttccttgtatgtcagaaaacccaagctgaaaatattacatttcttaaaacttctatgctcctgatctttttcttcttttctgttgtgccagaggcatgaactttatgcccccagcaccagttaagaagatgatttattaaacagacttaaatgaaagatggcttggtgtggatacacttagattcacagaccgtgccttggggcagttttagtgccaactttctaactaattcagaaatgaaaaacttctcattatttcaggataaatgtctaaacctaccagctcttgtctgaatgacataaaagtatcagcactaaaaatggagattttgttgttcacatgtcatctagactctcaaccctacaatgtttaacatatgagccagttacaaattaccaactaatggtatcttttgggcacttccaggtaaagcctcccagtgtccattgtatcaaactctttccctttcatacagggttacctgtacagtagtatcactcagaagttatgctggaggaattgctttcaattttttcattaggttcataaaatctactcagaaaatagatttaaaacacaaatgttaaaatccatgcaaaaacacaaatattttgatttgatttatgcaaagccctaagcctgtgctgtgcacagagaagagagcaatggcatgactacttgtctgtttactctcagaatgtgcatatatgcatttcatttccttgatttgaccctaattcaaggggccagtctgaagagtcagcaatgttaatttactagatctcaaaagtaagtattcatattactgcaaaaagcaagatgtcattttctcatcatttctgtgaatagaaaagctattttccaacaatagggatcccttataatagggaaatacttaactggtactgaactcagaaactgcagtgttctgcttggcttcattgattttatcaaaggacctctttatcctgagcaggtaaagctcaatgaattgaaatagtccagaaatacatgaatagctgtcctctgacagaaagtaagtttaaattgtaagaaaattactttatttccaaggattcccgagattcttgttcctgattatggtccaaaattccacacagatttgttcttgattcatttcagagtagtcagaaaaggtactgttctccttacatagagaaagaacatcctgtggtttcatctcagaactgtagctctcatatttgcaacagaaaaaagctggaccaacagcacactaatggctttttgtgaacccatcagaaagctaaagtcgaaggataatagtcttcctgaaatctagagagatgtggggtacctatgtaaaaattagagggctgtggtggacacaggaatcataaaatcagccagtccttttgctgaaatacatttctagtagtgccatgggtgatttgaaaatagtcttgttccttttcttcattcccttgcacactctgtctcctcttctccatggctttataaattacacacagaattaaggcttcccatttaggagaacatccatttctctctgacaacgtcatcaaagaagtgttcttcttccaagattttctcttgatgcagggaagtggcaaagttctagaagatcatcaagggctggaaatattgctgtggtcattccagagaaatgcaatcttaatattatagtcctatccaccattcgttgcctgggtttcaaatccaaataagcatggtggttgctatagtgacaatatgccacttttggaacctggagcttagtactactaggtacttatgagcttcataacgtcagtacttcctcccacactctgaatcatagctcagattttataacttcacaaaatgtaattccattctgtcctatatgagtcaattttattttagcagtatagaatatatgtcaaaagaatctaactcacttaacatgctaaatatacatactcaatatacatttaattaatagtaaatatattggcctgataagataaattttgtgcaaccattggaattcactgatttattattgaaactgggcaagattcacagctaattctttagcttacagttgttaaaataggattcctaccacacttcatttaagaagaaagtttgaaattctaaaataatgaatttcatttatggcagactgacatattttcattttactcaggaaccattcctaataattaaagactaattattaatgatctccaagatggtagcttgttgctagcaaaatgctaagaaaaaaatatcaatctcaaattacagtgcatttctagaatattaaaaaaaaaaaagtcagagaactggaaaccctcatacatggctggtgggaatgaaaaatgatgcagccactttggaaaaagtttccgtttctcaaaaagttatacatagaactaccctacgacccatcactttcattcctaggtatctacccaagacaaattaaaacatacgtccacataaagacttgcacatgaatgttcacagcattattcataactcgaaacgacctaaatgtctgtaaactggtaaatgggtagtgtttcatcctgccgaacccacgactggggtcgccctctaagagttcattaaaattaataaggt

SEQ ID NO: 18804 - RNA, 13181 nt, Homo sapiens
  source 1..13181: mol_type = other RNA
tgatggataaaagactacatattgggtacagtgtactctgctagggtcatgggtacatcaaaatctcagaaatcaccactaaagaacttatccatgtaagcaaacaccacctgttccccaaaaactattgaaataaaaaataataacaataaatatctttaaaaatatgactctatttaaatgttgagataaaatgaggctctattttccacgaagaaattaataatgctaaaattaagaattccagtttctccaataaacaattatatatttaacaaaaagtagtttattaatcacctttgttattgctgatatttatcccattgatttagaatcactactgccttcctgagagctaaacatctctttaatcaaataacatttttattttttgcttattatttgaacatgtgccttaaaagcactgcctattttgtttctaataagatatttatttttacctattttttacattgcagatttgttccactgttgttgttgtttttgtttcaggtatagaatgccacatactacataaaatgattctttttgcttatgaataatgtcaccaatttttaaaataacttgcagaaaacaaaactatgactaggcgttttcagtaaaaatgctaacattttggcaactttgtgaaattgtttattcctcctgatggtgtatacaacagagaaatgtggagaaaatgttctactaagaactcaatgataatttgctctacctatcacattttttaaattccatgtggttgtctccattaacggatggttaaacagctccaatttgaagacaaaatctttgattttttaggaaacaaatttttggagtatcagataatcattagttttcttatgacttgcaaaaaatttaccttggttatagtggtagctagggtcagacagattaattatattaaggctagacagtactatttttgaaggtagtttctcttcccttttaatagtaatgaattatttaaacaggaatcatgtaactaacacttagcactgttctaagaactttccgtatattacctcaattaattatcatgtaaatccagcaagttaataacttttaaaactcctattttacagataaacaatttgtagcacaaagagataaacagcttgcccaaagtcacacagctaggaagggggatcccagaattaaaactcaagcattctgcacttaaaattactacacaatactggcccactagcttaccatgttccatggcagaatccaatcattttacccacggccattctttaataatggcttcgaacttcttactccatgacctttgctgcttattttctcatgcacaccacagaccacactggactcattccttccacaagaactctgccccttgaatagagaagagcttttaaaatcgtaagtcaggactcacatcttctctataatattctccctaagtgtagtaaaccattgaaatgttcaatattatatgcctattctaattacttggagtagttgtcaataatacagtattgagaaatatcttgagaaaaaaaactagccttactagataagtgcttgatcattagcaacttttgttctgaccacagaacaactcatagcaagctgtaagtttgttccccctgctactgaaaccaatgccaaagtatgaaatatgttaccttgctcctaaaagcaatgagacataaaatagttggcttaataataacattaaaaaattctatttaaaagcaagctatacttcattatccccatcttctgatttaatatattagataggcatttatctataaacttacttgatcaaatatttgagtgaccatgatacccaaggcactgtgctggtactgcagagaatacagggccgaggaaatgatcttgtactcaagtatagaaagcagaacactttttttttttgtgaagatatgatggttacagtagtatgactgttagatgcatgaactcagataggacagacatacaatcaaccacataaggcagaaactgataaatactaaaagaaaaaaaaacaaatattaggcagaaatgtggaatattattgaatcatatattcaaatataataattaaaataaatctaacataagaataagaatgtgagaggatgcaatgtgggaaactacttaaagcttgaggagataacatgtatcaataatgtgaacaagagcatggagggaagcccaagccaaagaaagcaataagcactgcatgggcaaggagaatcaggaagggaagctcccccagcctgcagcagagtggtgcctaactagtgatttgtgaagatggctaaaaggaggaggtgtgctgtgagagggcagcgcaggcacaggcacttgcaccatcaatgacatcttgaccctacagagccaaatggagatgggcgtccagctcccaggaggtggatttgtggatctaagcctcatgttacttctcagctgaattgaaagaaacagctacaaatccccaaagtacaaagagatgctaagcaagaacaggtgttcttgtggccagagcatcaaaagcaacacgtacctgtcatgtcccacttgaggagaaactagttctacttgtatgcaagtatgtgagtgataaatacataaatggttatgaatgctaacaaagtgctgtttattggaatttggagtctcagaaattggctcttcactcaaagatttcaaaataatgcactcctgcttttagttagcattaactatattttttatcagttggaaaatagctacctatgtaatagagaacatcgaactgaagaaaaccagagaagacttcataaaggaaagttctctcccattttctccctcctgctaaactgctccaacccctttctcactttcttccaaaatacaaatgtcctcctaaacagccctcttttctgagttgcagatcaaatgtctggaaatcctccatctgcaggtgacaatgttgaaagatctagcaaggccttctcctcctgcaacattccatatatgaactaatgatatcaccacttctctgctgccatttctaaaccacaaggcttgcccagggcctctcaaaacccactgtccatgactgtatctccacttattttcccttagctaaaaatgtgttctcccctgaactgctttccctgtgccccttgtatcaaggttgctcattcttttcatcctcatatatttaagggtaaggagttcatatcagtgtcttcttcattccccatagtaccttctcaatcattcccaccccaatgtgtttgtaaaaatctatacctctctgaatctggtcccatttttctgtacaacttattgtggacatctgtgagttaccaacacagcattcattctatcatgtgcccttgttaactatacttcaatttttttcaacagtgacccatccccctacttatgccctaaagtcaactttttgataaactgactttagttctacctctagaattagtgtatgcatttacctggccacattgatggccttaggcataatcttatcagagtgaagctcaaaacttttgttcagtggttgcaggaaatggacactttttcttccacgagaggcaaactaggaagaatggattcaccattgctgctgatacctgtcttgcaaccaggaggaaaatcagcctaaagaaaaaactaacatataaaggaaagaagaaccaaagaaacaggaaaaaagaaaatgtagaaccaagacctgattgaatagttcctgaaacaactttacttgtggacttttctgtttgtctttaagtcacttgagatgggttttctgtactttcattgactttgtcatcactagaaactgttccttttcaaattcctactttaaaaatcctatcctcagacatcagcctcctgtcctttcagtttgttcacttacacatactacagtactaattagaatgtcatatctgttgaccatttttactatccacctactccttcctattttcatatataagttttgttcaccagtgggccaacccatgtagctcagtgtcttacatttagtaggcaattaataaattgtgttgattcattggttaattgattgttctctttgcctttctctctcaccccttcccaagtatgcttcacctagtgattattcttttaaattttttccataattatttttctgtaacacaatatatccttattactgtcccactggaaatcttcaataacactcattttgtccatagctggacctcagatgtggtccacactatgttcctgatgttgttgctttctaaaggttatcatcttccaattgagattgaggatggacaaacccttcctgaaccaaattcagtgctggaagccaccttaaaatgtcaacttcaaatatggtctaaaataatgtacttttaataaataaatataactctccatcatcacaaacctcagaaaagccatgcaatgatctctcctgcagtatctaattttgtaagaattccattctagacattatgctttaatggaacactggcaaaataaaagttatccaaagagtaaccaggatggtgaaaagcccagaaaccatgtgtcaaggggaaaacagggtttctttgcagagagagggtgtggggaccataacatttatgttctgatatttgaaggactgtcaagtggaagaacaaaagttgcaattctcttctgctccagacatcagaaaaagattaaatttaatcttatatggagttatatcttagctcaatatgaaatgtaacattaaaataatgtttctatccaggtatccagctataaaaggggcttacataaaagcagagttttataaagtatcaatcaagttagtctagtttgtgctgtagcaacaaagaacccccaaatctcaatggtatatcaaaaaaagtttgtttcttatttatactactttatttgtccagcacaggtcacaaaagatcctacgcattgtagccttcaaagactcaagatgacagaagatccaccatcctatgacactgccatctaaacacaagtctccagcggccactgtggcaaggaaacagagcttgaatcataaatcagctcttaaatgcttctgcctggaagtgattcacatcacttcacttaaatttcattggccaaagcagtccatggccatgtataatttcaaggagatgagacagctgtaaaaggaaggatgtcagaagcttcagttagcacttggaacatctaccataactttcagtaggatttaagcagaattcaaattctcattaggaatatcatagaaaaagttagattgctaagcctctttaaactctaggattctataattccaaacttatgtcagatagttcctttaatatcagggattttgcttcctagggtaaaatgaataactctggagcactgaaacttcccatatacaaaggactatgctcaatatttgaatttactgagctgagcttacaaagacttggcttggaagagctaaatattggcaggtcaacagccctaactctgtaagcttgttatggtccatttttttcaaacattgcttcaaatatttacatttgacttttacataaaagttgctgattttcagtagaggctgagatgaacgacagttgataactgttcctcatgttctatagaatttatgtgtaaggtttccagctatttttctatcttccttggtaagactgtagtgtagctaaacaggtggacttaaatgtcagctgtattctagtggcttaataatgcctttgaatacgtaatagccaatgcttacaggttatgttattttatattacagtctcctgtttaattttactgcagatacgtcttaaattgagagcaattactcccttcatttttgccattttaaacctgctgtgtactcattttttttaaattatgggccaaaaaaggacagctatacattttcagtgtcatggatctagagttatagctctagaggggccacagagatcacctagtttgcccctttgttttacatacaaaaaatttaagaacagttaacatttgttgagagtgtaccatgttctgggcactggcctactgttttctcatgtattaactcaactgatcttctcaatagcccaagaaaataaatactgtcatcatctccatttcacagatgaataaacttacctaagattgggaaacatttcccccttattagacaggtcaatattttaaaaaaaaaaatggcatagcctggtgctggggagaacacgaacaggcacatggcctcatttactgttcagcattttgtgacatttagctcaaactttttgatattgaatcttcctccatttctccacagttcttacatatcaatttggacaaaggtgacaagataatagcaaattccaagaaaaactattacatagttcaaataatcacacaattacatattagacagaaagtaaaggctagagaaagtctgcagcactacctaatctgagaaaatgattgggaaggaatgttaaaattattaaccattgaggcttgggccctaggctcccttactgggaagtttctggaatagtttctagagttatgtctgaaatagttttccaattctgattgaaacctttaagctaataatgcttacctatgaatgaagagatttgggtgacttttacatttttctttgtacttttcaatattgtttaattttccattgcagtgacaatacattttataaaatcatcgagaagatttaaacaaatgcaatgagtttattgaatgagctgaactcaggaagatagcaaaaagcaactttgttctttctcaccctgtacctgcatacctgttctttgggtttcatttaacaagctattctacaacctaagagataggcactaccctcccactcctgaggtctaccacttttagaactgtctactattgtcaacactacctgcgacccagtcttcggcatcccctcctcaaactcatccccctaaagttccagtctctgtcctgctcagacacctgtgtcagggctctctccagtgattctgaattgagtgcccttgggcacccctggtaagagcctctgtctactcaaccacacccagagctaccattcgctgtatgaagctggaaaagttcacaccccttagctctggtgctgaagtggacacgggtagagcacaggaaaatgtgctccctacatcccaaatgaaagccctgaactaatagaaacaaatgatgaggaggctctgtatcactgaagtatggacacattgtgggttaaaggctttggcagactgaactggagacataaccttcattcatcacacaatttctatagaaaaatgtgtcgagttcaaaacaactgacctacaaatgatccttaggaacataatttgtctggaaactgggggctgcttttataaccatctccagcctgtcagatccaatagattagagtcaagacagcacctttgatttacagtcttggccctgttgctgaagcacttcctaattcacactctctattcttaaaatgagaggcataatatgtctgctccaactacaaggttgttgagataataagcatggctatttctgagaaaatatcttacaaaattgacaatataagtgtttactattatttcatgtggtgcattacagaattcacagtacaggtaattggttatagggaagtcgtttctgagattaataagactgccgcaaaagtatcacaatatgctcctgttttttccccattcctgatttctttccttagcaaaaaatgttcctttgtctttcttaacctatgcatttttaggttattggcttttagaatattggcattactgaaaccctgtctaactttaggagcgctaattgagtatataataacacacatgtaaatcaacaaattttagaaagccttagaatctgcaaaaagcatgaaacataatttatcctatgctaagtacagtaactaggtaatgccagtgttaaaaaaaaaagtataaaacttgaaaataaggataaaagggtagagcaagcccttttgatgtctactggtatattatttcaatagtccacttcatgacaatttatctgattactcatgtttgactttgctatttcctatttgattagagactagacactatggaattatatgttaaattgtagatttttgttaagtaaaaaagataaccttaaagatggctgttctgttgtcccgtgggccactaaccaatgttgtatccaacccagctatcctattctaatatccttttaatgtctttcctgctgtactatatatatcattgttccttaaatgctcttggaaccagtttcatcctcatattggtatgtatgtatatgtatacatatatacacatatatgtatatatgtatacattatctgtaaacataataaagtgctttgaagaaattttaaaaataggaaagtgggtggtgccaaggaagctgagggaagaaaatgtttgagaagggaatgctcagaagaggctgcactgccataagttgaagggacttagcagtaaggaataggtcagtaaccttggagagagcagcattcatggggtggtgaaggcagaaaccgcatcattaagagcaaggggaagagggccagaacgtacacaccactttagggaagttggaatgtggggagagcagtgcaatgagatggtgccagatagataagagatccaaggagaggtatatattttgtgtgttttctgggttttttgatgttgtttgttttaatgggtgagaccagagtatatttaaatgcagatgggaagaacagtttgaagatcaagtaagagggatggaggtgggggtgaataattaaaagaaaaaagattcctgaggaggcaagaggggatagaatcccaagaacagatatttcagggtgggggcggggctggcaacagacagcatgttggctggctgaagttacggtgggaggtggtgggagttgtaagtctgaggagcttgtgaaatgtttcagatggaagctgtgggaaatagaagaaagctaaaaaacacacatgaattgcaaaatagcattgaggaccccagtacaagttgaatgcaatgacatcatagtggcaccaatatgattatatgaggtttttttttctccagccatgctcaagacttcagcttagccaaggaaatagcaggcacggtaggtattttctggctggttatgagtggaatataatgagagaaggtaaataggacacttatagggaggtaactgaagcaatggactaagcacttgtccaaacatttttgttctcatgctctcaaaagattttggaaaactatttctcacatattttgaaatcaaaatctaaaaatttttaacacataaagtgaaatagtttcaaaggatgtatttatggcttatattatatatgtacattaaatatatttttatccaagtcttggagttgtagatttagctcattctatttatagaacacgtctttcagataatcaggccacattgtgaaactaatcagccaaatcagggttacttttcatcagaaccagtacaattttattttaaaattcatacagtcatgcatctgtggaatacttctgtattctaagataggttaattgatttttaaatggatggttgattgttgggtagatagctggtggatagatgaataaaacaagacatggatggatagacaaattcttatcttgagtttgtctcctggataaaacaagatcccctcaaatatttctctctgaagtttttttttattttactttcaagagactttccctcaagaaagtggtattctagatttgtccctctttttgatgccccaagtgtttttacaccctggagcaatgcatcaaaatacaacttaggatgggggaagtacacttttcttttgtaaagtggagaagggcaatgtgaaaggtgaaaaaggaaagactaattggtagacatcagagtttgtatgcaggtcagcttgaagaatgaatatgaggaagttgagatttagaaatttctacactacagctttctaagcttttttgattatcccacaggtacctaaaacttaacatgcctaaaattgaacttacatatctacctcatcctagtcctccttcctcagtgagtggcaccatttctattcattaagacaagacagaaacctggcagtcaccctgaacttcttgttctctcatgcccttcatatccaactaaacaccaagatctggacattttttctcataatgatctcctgagtcagcccacatccctctatccccatggctatctctctgctgcagggtatggttgcctctcactcagctgccaaaatctgcctgtctctagtcttgagtcctctccacctgctctccatactacaaccagagaaagtattctaaaacatgtctgactaaatagctccatttttaaaaagttatcaatgacttcctataaccctaggccttattattcacttactagattactatttcaatcaagctctaaggacaaatcctaaactcattggcatggctttcaaggcccttctgaacttggcctctgctcatcatggcagcttccgctctccccactccatactctgcttatgaagtgttttcatcccaagtctcaccaggctctcctgcctcaaacactctttctgcctccttcttctagctccctcctatttagcattaaggtttcagctgagatgtaatttcctctagaaagcttttcctaatccctcaagtttgggtttgatccttatcttacatacttctgtgacgcattgtttgtagtccattatagcatttactctacattgagttttaactgtttacatgtctgaatacccaagagcagagggacatatgtgtgtgtctattcacttttgtattgtcagtgtctagggtactagccactgcctggtgcagagtaggtatccaataaacacgtacttaccgaataaatacgtgaagctaccaaaattttgcccccaaaataaatcacattccttctatgagtggcttataaacctgtttagtgaccaaatataaagttttcatcaagttcatatgaaattgttggcaaaaaataatccataagcttgatggggaaaaaattccatgccccatctctctaacaatgatatcaaaaactacttccttatacatagcaaaataacttagctgagaactgagtcaaaaggaactgaaattttcattattttattaattcattcaatgatcaatggtcacttagctctgccttcatgaagcagtgttgctctagtctagtctaatgcttgccccatgaagcccactgaaccctggagaaaagctggcccatctcttcagctttccaaattttattatatagaactaggagcagctgcttttatccaagtaggaataatttttaaatagcatttttccttgtatgtcagaaaacccaagctgaaaatattacatttcttaaaacttctatgctcctgatctttttcttcttttctgttgtgccagaggcatgaactttatgcccccagcaccagttaagaagatgatttattaaacagacttaaatgaaagatggcttggtgtggatacacttagattcacagaccgtgccttggggcagttttagtgccaactttctaactaattcagaaatgaaaaacttctcattatttcaggataaatgtctaaacctaccagctcttgtctgaatgacataaaagtatcagcactaaaaatggagattttgttgttcacatgtcatctagactctcaaccctacaatgtttaacatatgagccagttacaaattaccaactaatggtatcttttgggcacttccaggtaaagcctcccagtgtccattgtatcaaactctttccctttcatacagggttacctgtacagtagtatcactcagaagttatgctggaggaattgctttcaattttttcattaggttcataaaatctactcagaaaatagatttaaaacacaaatgttaaaatccatgcaaaaacacaaatattttgatttgatttatgcaaagccctaagcctgtgctgtgcacagagaagagagcaatggcatgactacttgtctgtttactctcagaatgtgcatatatgcatttcatttccttgatttgaccctaattcaaggggccagtctgaagagtcagcaatgttaatttactagatctcaaaagtaagtattcatattactgcaaaaagcaagatgtcattttctcatcatttctgtgaatagaaaagctattttccaacaatagggatcccttataatagggaaatacttaactggtactgaactcagaaactgcagtgttctgcttggcttcattgattttatcaaaggacctctttatcctgagcaggtaaagctcaatgaattgaaatagtccagaaatacatgaatagctgtcctctgacagaaagtaagtttaaattgtaagaaaattactttatttccaaggattcccgagattcttgttcctgattatggtccaaaattccacacagatttgttcttgattcatttcagagtagtcagaaaaggtactgttctccttacatagagaaagaacatcctgtggtttcatctcagaactgtagctctcatatttgcaacagaaaaaagctggaccaacagcacactaatggctttttgtgaacccatcagaaagctaaagtcgaaggataatagtcttcctgaaatctagagagatgtggggtacctatgtaaaaattagagggctgtggtggacacaggaatcataaaatcagccagtccttttgctgaaatacatttctagtagtgccatgggtgatttgaaaatagtcttgttccttttcttcattcccttgcacactctgtctcctcttctccatggctttataaattacacacagaattaaggcttcccatttaggagaacatccatttctctctgacaacgtcatcaaagaagtgttcttcttccaagatttttcagtatcatgctcactagctgggtgatgggttcaactgtactccaaacttcagcatcacacattatactcttgtaacaaacctgcacatgtacc

SEQ ID NO: 18805 - RNA, 2713 nt, Homo sapiens
  source 1..2713: mol_type = other RNA
tgatggataaaagactacatattgggtacagtgtactctgctagggtcatgggtacatcaaaatctcagaaatcaccactaaagaacttatccatgtaagcaaacaccacctgttccccaaaaactattgaaataaaaaataataacaataaatatctttaaaaatatgactctatttaaatgttgagataaaatgaggctctattttccacgaagaaattaataatgctaaaattaagaattccagtttctccaataaacaattatatatttaacaaaaagtagtttattaatcacctttgttattgctgatatttatcccattgatttagaatcactactgccttcctgagagctaaacatctctttaatcaaataacatttttattttttgcttattatttgaacatgtgccttaaaagcactgcctattttgtttctaataagatatttatttttacctattttttacattgcagatttgttccactgttgttgttgtttttgtttcaggtatagaatgccacatactacataaaatgattctttttgcttatgaataatgtcaccaatttttaaaataacttgcagaaaacaaaactatgactaggcgttttcagtaaaaatgctaacattttggcaactttgtgaaattgtttattcctcctgatggtgtatacaacagagaaatgtggagaaaatgttctactaagaactcaatgataatttgctctacctatcacattttttaaattccatgtggttgtctccattaacggatggttaaacagctccaatttgaagacaaaatctttgattttttaggaaacaaatttttggagtatcagataatcattagttttcttatgacttgcaaaaaatttaccttggttatagtggtagctagggtcagacagattaattatattaaggctagacagtactatttttgaaggtagtttctcttcccttttaatagtaatgaattatttaaacaggaatcatgtaactaacacttagcactgttctaagaactttccgtatattacctcaattaattatcatgtaaatccagcaagttaataacttttaaaactcctattttacagataaacaatttgtagcacaaagagataaacagcttgcccaaagtcacacagctaggaagggggatcccagaattaaaactcaagcattctgcacttaaaattactacacaatactggcccactagcttaccatgttccatggcagaatccaatcattttacccacggccattctttaataatggcttcgaacttcttactccatgacctttgctgcttattttctcatgcacaccacagaccacactggactcattccttccacaagaactctgccccttgaatagagaagagcttttaaaatcgtaagtcaggactcacatcttctctataatattctccctaagtgtagtaaaccattgaaatgttcaatattatatgcctattctaattacttggagtagttgtcaataatacagtattgagaaatatcttgagaaaaaaaactagccttactagataagtgcttgatcattagcaacttttgttctgaccacagaacaactcatagcaagctgtaagtttgttccccctgctactgaaaccaatgccaaagtatgaaatatgttaccttgctcctaaaagcaatgagacataaaatagttggcttaataataacattaaaaaattctatttaaaagcaagctatacttcattatccccatcttctgatttaatatattagataggcatttatctataaacttacttgatcaaatatttgagtgaccatgatacccaaggcactgtgctggtactgcagagaatacagggccgaggaaatgatcttgtactcaagtatagaaagcagaacactttttttttttgtgaagatatgatggttacagtagtatgactgttagatgcatgaactcagataggacagacatacaatcaaccacataaggcagaaactgataaatatttatttccaaggattcccgagattcttgttcctgattatggtccaaaattccacacagatttgttcttgattcatttcagagtagtcagaaaaggtactgttctccttacatagagaaagaacatcctgtggtttcatctcagaactgtagctctcatatttgcaacagaaaaaagctggaccaacagcacactaatggctttttgtgaacccatcagaaagctaaagtcgaaggataatagtcttcctgaaatctagagagatgtggggtacctatgtaaaaattagagggctgtggtggacacaggaatcataaaatcagccagtccttttgctgaaatacatttctagtagtgccatgggtgatttgaaaatagtcttgttccttttcttcattcccttgcacactctgtctcctcttctccatggctttataaattacacacagaattaaggcttcccatttaggagaacatccatttctctctgacaacgtcatcaaagaagtgttcttcttccaagattttctcttgatgcagggaagtggcaaagttctagaagatcatcaagggctggaaatattgctgtggtcattccagagaaatgcaatagatgtgactgggcgcagcggccaccgtaaggcgtaaggggtgccaagtgccggttccagtcccgcccag

SEQ ID NO: 18806 - RNA, 76 nt, Homo sapiens
  source 1..76: mol_type = other RNA
tgattgtccaaacgcaattcttgtacgagtctgcggccaaccgagaattgtggctggacatctgtggctgagctcc

SEQ ID NO: 18807 - RNA, 1692 nt, Homo sapiens
  source 1..1692: mol_type = other RNA
tgcaaaagtaatcacagtttttcacactggtccaatggaaatggaagaaacaaacaactccatggatttcactccttctctgagaggtcacctgtcaatgacagaactagaaacctggaattccacagaaacctctctcctaagctgtgagatcccagtgagcagagctggccactacaaatcacagagttgagcccaagtctttcagctattcctcccagggatttacaacaagtggagagtcaggaatcctaaccgaggagggtgtggaggtggtgggaattgcatttgcattatttacagattagcctagcacagcaaatctgccctctcagcagaggtgacccaaggcattatatgaagggcaagttgctgacccagaaaagggtgacagcggcaaggcgctaccactaaccaaaacacaaacatgggtaaatggaatagagtccaagctccggcagctgggtcatactttggaatggcccttcattccctcctcacccccagcctcccacccccaatgccaccgcttttgaacacctatgacatttcacattagaatatgatcttggcagcaagtggaggggaaagccggtgatttccaggagttcccttctgaggtctaactgagcctcctctggctttgggacagcagatctaagtacattttggacctcaggaacctggggtaagagtctttctccatgaggctgtgtacttttccttgggcttggtcaaagcaagtcagggatggctcctgcaggttcttcctcgtggcttctcgggtctggaagtcaatgtttacctcccgtggagcctgcacatccacaaactcctcaaagatcctatgggccttagagaccagttttgcagttgacctggtcttcttgaactcctcacaggccaaccagaattccaggttctcctcactgaactccgtcttcaagaaggcacggaatgcagccaccccatacttatgagagagaagcacatcaaaggaatctgcccacctcgtagcttcttctgtcgataatctcttgagagcgcggttgggtttgtctggaagaatagctgtgaaatcactacacgagtctgacttgtgagacaggcatcccagtcgagtcctcatccctttgttcctgcgtggcatcagtaaggccgccatacaggcatcagcttacggttaacccttgggctggtatgcagggacgtcagggcaggaaataagactgcggggctcaggaatttacccttgcacgtcctctcactgtctttggccagtcctcatggcctgagggtctttgccaactggatggtcagagaggcttcgggttaaggtgttccacatgggtcttcacactgcctgcttcagttccagaaggaggactctcttcctgcttgccctagtgtagtggttctccaagcgtggtccctgaaccagcagtgtcagcatcacctgcctggcggtgggcagcgcagctgggaaggtgtggctggtgcgggccccagctgggcatggttcggtgaggccctgagtgatagagtcagccacctcctcctggcacctgggagagggtggcagagggcagcccacttcacccagcgcccctagaatagcggctgcaacatgctgctcctgccggctccgctcctctccaggctctgcatctcatgaaaagggaaagagcgagt

SEQ ID NO: 18808 - RNA, 1581 nt, Homo sapiens
  source 1..1581: mol_type = other RNA
tgcaaaagtaatcacagtttttcacactggtccaatggaaatggaagaaacaaacaactccatggatttcactccttctctgagaggtcacctgtcaatgacagaactagaaacctggaattccacagaaacctctctcctaagctgtgagatcccagtgagcagagctggccactacaaatcacagagttgagcccaagtctttcagctattcctcccagggatttacaacaagtggagagtcaggaatcctaaccgaggagggtgtggaggtggtgggaattgcatttgcattatttacagattagcctagcacagcaaatctgccctctcagcagaggtgacccaaggcattatatgaagggcaagttgctgacccagaaaagggtgacagcggcaaggcgctaccactaaccaaaacacaaacatgggtaaatggaatagagtccaagctccggcagctgggtcatactttggaatggcccttcattccctcctcacccccagcctcccacccccaatgccaccgcttttgaacacctatgacatttcacattagaatatgatcttggcagcaagtggaggggaaagccggtgatttccaggagttcccttctgaggtctaactgagcctcctctggctttgggacagcagatctaagtacattttggacctcaggaacctggggtaagagtctttctccatgaggctgtgtacttttccttgggcttggtcaaagcaagtcagggatggctcctgcaggttcttcctcgtggcttctcgggtctggaagtcaatgtttacctcccgtggagcctgcacatccacaaactcctcaaagatcctatgggccttagagaccagttttgcagttgacctggtcttcttgaactcctcacaggccaaccagaattccaggttctcctcactgaactccgtcttcaagaaggcacggaatgcagccaccccatacttatgagagagaagcacatcaaaggaatctgcccacctcgtagcttcttctgtcgataatctcttgagagcgcggttgggtttgtctggaagaatagctgtgaaatcactacacgagtctgacttgtgagacaggcatcccagtcgagtcctcatccctttgttcctgcgtggcatcagtaaggccgccatacaggcatcagcttacggttaacccttgggctggtatgcagggacgtcagggcaggaaataagactgcggggctcaggaatttacccttgcacgtcctctcactgtctttggccagtcctcatggcctgagggtctttgccaactggatggtcagagaggcttcgggttaaggtgttccacatgggtcttcacactgcctgcttcagttccagaaggaggactctcttcctgcttgccctagtgtagtggttctccaagcgtggtccctgaaccagcagtgtcagcatcaccttacatcctagcagccacaggagtcggcacatcaaccggtcctgctccagaatggccagtaattcaagacccggccacagacgagacacaggtggttcctgtcaggaacagcatttcctggtat

SEQ ID NO: 18809 - RNA, 2197 nt, Homo sapiens
  source 1..2197: mol_type = other RNA
tgcaaaagtaatcacagtttttcacactggtccaatggaaatggaagaaacaaacaactccatggatttcactccttctctgagaggtcacctgtcaatgacagaactagaaacctggaattccacagaaacctctctcctaagctgtgagatcccagtgagcagagctggccactacaaatcacagagttgagcccaagtctttcagctattcctcccagggatttacaacaagtggagagtcaggaatcctaaccgaggagggtgtggaggtggtgggaattgcatttgcattatttacagattagcctagcacagcaaatctgccctctcagcagaggtgacccaaggcattatatgaagggcaagttgctgacccagaaaagggtgacagcggcaaggcgctaccactaaccaaaacacaaacatgggtaaatggaatagagtccaagctccggcagctgggtcatactttggaatggcccttcattccctcctcacccccagcctcccacccccaatgccaccgcttttgaacacctatgacatttcacattagaatatgatcttggcagcaagtggaggggaaagccggtgatttccaggagttcccttctgaggtctaactgagcctcctctggctttgggacagcagatctaagtacattttggacctcaggaacctggggtaagagtctttctccatgaggctgtgtacttttccttgggcttggtcaaagcaagtcagggatggctcctgcaggttcttcctcgtggcttctcgggtctggaagtcaatgtttacctcccgtggagcctgcacatccacaaactcctcaaagatcctatgggccttagagaccagttttgcagttgacctggtcttcttgaactcctcacaggccaaccagaattccaggttctcctcactgaactccgtcttcaagaaggcacggaatgcagccaccccatacttatgagagagaagcacatcaaaggaatctgcccacctcgtagcttcttctgtcgataatctcttgagagcgcggttgggtttgtctggaagaatagctgtgaaatcactacacgagtctgacttgtgagacaggcatcccagtcgagtcctcatccctttgttcctgcgtggcatcagtaaggccgccatacaggcatcagcttacggttaacccttgggctggtatgcagggacgtcagggcaggaaataagactgcggggctcaggaatttacccttgcacgtcctctcactgtctttggccagtcctcatggcctgagggtctttgccaactggatggtcagagaggcttcgggttaaggtgttccacatgggtcttcacactgcctgcttcagttccagaaggaggactctcttcctgcttgccctagtgtagtggttctccaagcgtggtccctgaaccagcagtgtcagcatcacctttctcatttccttttgttcctcttgagcattcatttgtctcctcactgctcactgcagggttttcctcttgccagcctcttttctttattcactactttatactcccccttctaagtgtgtcttgacctggccatggtgagatgtgggccacactacacactctactgcccactcacttatcacctttccagtctaacacacacttctttcaggaaacctgctctgcctggcggtgggcagcgcagctgggaaggtgtggctggtgcgggccccagctgggcatggttcggtgaggccctgagtgatagagtcagccacctcctcctggcacctgggagagggtggcagagggcagcccacttcacccagcgcccctagaatagcggctgcaacatgctgctcctgccggctccgctcctctccaggctctgcatctcatgaaaagggaaagagcgagtgagcggcaggggagggggtggggaagcagagggaggggagaggggcactctgacagatgatgcgcactgccacgcagagtcgggggaggaccgcaggctccagcaggatggcactgcctgtgtggctctcccgctcccagctcgctcacagacagctgcctccgaggggctggtggctctccagaattcagggagaggcagagttcagaggggatggcagaggggaaggtgagggagggaagagatcacctgggacacaaggaggcgaaacggggtaact

SEQ ID NO: 18810 - RNA, 1418 nt, Homo sapiens
  source 1..1418: mol_type = other RNA
tgcaaaagtaatcacagtttttcacactggtccaatggaaatggaagaaacaaacaactccatggatttcactccttctctgagaggtcacctgtcaatgacagaactagaaacctggaattccacagaaacctctctcctaagctgtgagatcccagtgagcagagctggccactacaaatcacagagttgagcccaagtctttcagctattcctcccagggatttacaacaagtggagagtcaggaatcctaaccgaggagggtgtggaggtggtgggaattgcatttgcattatttacagattagcctagcacagcaaatctgccctctcagcagaggtgacccaaggcattatatgaagggcaagttgctgacccagaaaagggtgacagcggcaaggcgctaccactaaccaaaacacaaacatgggtaaatggaatagagtccaagctccggcagctgggtcatactttggaatggcccttcattccctcctcacccccagcctcccacccccaatgccaccgcttttgaacacctatgacatttcacattagaatatgatcttggcagcaagtggaggggaaagccggtgatttccaggagttcccttctgaggtctaactgagcctcctctggctttgggacagcagatctaagtacattttggacctcaggaacctggggtaagagtctttctccatgaggctgtgtacttttccttgggcttggtcaaagcaagtcagggatggctcctgcaggttcttcctcgtggcttctcgggtctggaagtcaatgtttacctcccgtggagcctgcacatccacaaactcctcaaagatcctatgggccttagagaccagttttgcagttgacctggtcttcttgaactcctcacaggccaaccagaattccaggttctcctcactgaactccgtcttcaagaaggcacggaatgcagccaccccatacttatgagagagaagcacatcaaaggaatctgcccacctcgtagcttcttctgtcgataatctcttgagagcgcggttgggtttgtctggaagaatagctgtgaaatcactacacgagtctgacttgtgagacaggcatcccagtcgagtcctcatccctttgttcctgcgtggcatcagtaaggccgccatacaggcatcagcttacggttaacccttgggctggtatgcagggacgtcagggcaggaaataagactgcggggctcaggaatttacccttgcacgtcctctcactgtctttggccagtcctcatggcctgagggtctttgccaactggatggtcagagaggcttcgggttaaggtgttctcccaccacttgagccaggcagcaagcggccccactgaaagctcttctctctgcttgtcacatccagtaaatact

SEQ ID NO: 18811 - RNA, 1544 nt, Homo sapiens
  source 1..1544: mol_type = other RNA
tgcaaaagtaatcacagtttttcacactggtccaatggaaatggaagaaacaaacaactccatggatttcactccttctctgagaggtcacctgtcaatgacagaactagaaacctggaattccacagaaacctctctcctaagctgtgagatcccagtgagcagagctggccactacaaatcacagagttgagcccaagtctttcagctattcctcccagggatttacaacaagtggagagtcaggaatcctaaccgaggagggtgtggaggtggtgggaattgcatttgcattatttacagattagcctagcacagcaaatctgccctctcagcagaggtgacccaaggcattatatgaagggcaagttgctgacccagaaaagggtgacagcggcaaggcgctaccactaaccaaaacacaaacatgggtaaatggaatagagtccaagctccggcagctgggtcatactttggaatggcccttcattccctcctcacccccagcctcccacccccaatgccaccgcttttgaacacctatgacatttcacattagaatatgatcttggcagcaagtggaggggaaagccggtgatttccaggagttcccttctgaggtctaactgagcctcctctggctttgggacagcagatctaagtacattttggacctcaggaacctggggtaagagtctttctccatgaggctgtgtacttttccttgggcttggtcaaagcaagtcagggatggctcctgcaggttcttcctcgtggcttctcgggtctggaagtcaatgtttacctcccgtggagcctgcacatccacaaactcctcaaagatcctatgggccttagagaccagttttgcagttgacctggtcttcttgaactcctcacaggccaaccagaattccaggttctcctcactgaactccgtcttcaagaaggcacggaatgcagccaccccatacttatgagagagaagcacatcaaaggaatctgcccacctcgtagcttcttctgtcgataatctcttgagagcgcggttgggtttgtctggaagaatagctgtgaaatcactacacgagtctgacttgtgagacaggcatcccagtcgagtcctcatccctttgttcctgcgtggcatcagtaaggccgccatacaggcatcagcttacggttaacccttgggctggtatgcagggacgtcagggcaggaaataagactgcggggctcaggaatttacccttgcacgtcctctcactgtctttggccagtcctcatggcctgagggtctttgccaactggatggtcagagaggcttcgggttaaggtgttctgaagctcctctggctgcagctcagggagaagtccccacagcccacagctgcctccctctgcacccagaggctgtgcggggggcagcaaagaataggtattaactctttccagtcaccagtgagctaaaaatcaagtgtccaggggaccctcttctaatgagccccgctgctggctgaaggttggctgctgcaccgggagt

SEQ ID NO: 18812 - RNA, 1536 nt, Homo sapiens
  source 1..1536: mol_type = other RNA
tgcaaaagtaatcacagtttttcacactggtccaatggaaatggaagaaacaaacaactccatggatttcactccttctctgagaggtcacctgtcaatgacagaactagaaacctggaattccacagaaacctctctcctaagctgtgagatcccagtgagcagagctggccactacaaatcacagagttgagcccaagtctttcagctattcctcccagggatttacaacaagtggagagtcaggaatcctaaccgaggagggtgtggaggtggtgggaattgcatttgcattatttacagattagcctagcacagcaaatctgccctctcagcagaggtgacccaaggcattatatgaagggcaagttgctgacccagaaaagggtgacagcggcaaggcgctaccactaaccaaaacacaaacatgggtaaatggaatagagtccaagctccggcagctgggtcatactttggaatggcccttcattccctcctcacccccagcctcccacccccaatgccaccgcttttgaacacctatgacatttcacattagaatatgatcttggcagcaagtggaggggaaagccggtgatttccaggagttcccttctgaggtctaactgagcctcctctggctttgggacagcagatctaagtacattttggacctcaggaacctggggtaagagtctttctccatgaggctgtgtacttttccttgggcttggtcaaagcaagtcagggatggctcctgcaggttcttcctcgtggcttctcgggtctggaagtcaatgtttacctcccgtggagcctgcacatccacaaactcctcaaagatcctatgggccttagagaccagttttgcagttgacctggtcttcttgaactcctcacaggccaaccagaattccaggttctcctcactgaactccgtcttcaagaaggcacggaatgcagccaccccatacttatgagagagaagcacatcaaaggaatctgcccacctcgtagcttcttctgtcgataatctcttgagagcgcggttgggtttgtctggaagaatagctgtgaaatcactacacgagtctgacttgtgagacaggcatcccagtcgagtcctcatccctttgttcctgcgtggcatcagtaaggccgccatacaggcatcagcttacggttaacccttgggctggtatgcagggacgtcagggcaggaaataagactgcggggctcaggaatttacccttgcacgtcctctcactgtctttggccagtcctcatggcctgagggtctttgccaactggatggtcagagaggcttcgggttaaggtgttctggggaaaaagtagatctttcttttagcagtcaaatcctcggcgagtgaagggcatgtgtgcatgaacacataggggcacacacacacatatacacacacaggcatgcacaacacacctcccaccacttgagccaggcagcaagcggccccactgaaagctcttctctctgcttgtcacatccagtaaatact

SEQ ID NO: 18813 - RNA, 1525 nt, Homo sapiens
  source 1..1525: mol_type = other RNA
tgcaaaagtaatcacagtttttcacactggtccaatggaaatggaagaaacaaacaactccatggatttcactccttctctgagaggtcacctgtcaatgacagaactagaaacctggaattccacagaaacctctctcctaagctgtgagatcccagtgagcagagctggccactacaaatcacagagttgagcccaagtctttcagctattcctcccagggatttacaacaagtggagagtcaggaatcctaaccgaggagggtgtggaggtggtgggaattgcatttgcattatttacagattagcctagcacagcaaatctgccctctcagcagaggtgacccaaggcattatatgaagggcaagttgctgacccagaaaagggtgacagcggcaaggcgctaccactaaccaaaacacaaacatgggtaaatggaatagagtccaagctccggcagctgggtcatactttggaatggcccttcattccctcctcacccccagcctcccacccccaatgccaccgcttttgaacacctatgacatttcacattagaatatgatcttggcagcaagtggaggggaaagccggtgatttccaggagttcccttctgaggtctaactgagcctcctctggctttgggacagcagatctaagtacattttggacctcaggaacctggggtaagagtctttctccatgaggctgtgtacttttccttgggcttggtcaaagcaagtcagggatggctcctgcaggttcttcctcgtggcttctcgggtctggaagtcaatgtttacctcccgtggagcctgcacatccacaaactcctcaaagatcctatgggccttagagaccagttttgcagttgacctggtcttcttgaactcctcacaggccaaccagaattccaggttctcctcactgaactccgtcttcaagaaggcacggaatgcagccaccccatacttatgagagagaagcacatcaaaggaatctgcccacctcgtagcttcttctgtcgataatctcttgagagcgcggttgggtttgtctggaagaatagctgtgaaatcactacacgagtctgacttgtgagacaggcatcccagtcgagtcctcatccctttgttctgtctttggccagtcctcatggcctgagggtctttgccaactggatggtcagagaggcttcgggttaaggtgttccacatgggtcttcacactgcctgcttcagttccagaaggaggactctcttcctgcttgccctagtgtagtggttctccaagcgtggtccctgaaccagcagtgtcagcatcaccggttggtggtctttctgtaaggagctggcatcatctggtcattgcttgatttgtttcattcagttggtttcttttattgtgtccatcatagtagttaagcaggcaggctctagagccagactgccttggtttaaatcccagctctactattttaaagtgctgtgactttaggcaagtaataaccctgccgtgcctca

SEQ ID NO: 18814 - RNA, 1563 nt, Homo sapiens
  source 1..1563: mol_type = other RNA
tgcaaaagtaatcacagtttttcacactggtccaatggaaatggaagaaacaaacaactccatggatttcactccttctctgagaggtcacctgtcaatgacagaactagaaacctggaattccacagaaacctctctcctaagctgtgagatcccagtgagcagagctggccactacaaatcacagagttgagcccaagtctttcagctattcctcccagggatttacaacaagtggagagtcaggaatcctaaccgaggagggtgtggaggtggtgggaattgcatttgcattatttacagattagcctagcacagcaaatctgccctctcagcagaggtgacccaaggcattatatgaagggcaagttgctgacccagaaaagggtgacagcggcaaggcgctaccactaaccaaaacacaaacatgggtaaatggaatagagtccaagctccggcagctgggtcatactttggaatggcccttcattccctcctcacccccagcctcccacccccaatgccaccgcttttgaacacctatgacatttcacattagaatatgatcttggcagcaagtggaggggaaagccggtgatttccaggagttcccttctgaggtctaactgagcctcctctggctttgggacagcagatctaagtacattttggacctcaggaacctggggtaagagtctttctccatgaggctgtgtacttttccttgggcttggtcaaagcaagtcagggatggctcctgcaggttcttcctcgtggcttctcgggtctggaagtcaatgtttacctcccgtggagcctgcacatccacaaactcctcaaagatcctatgggccttagagaccagttttgcagttgacctggtcttcttgaactcctcacaggccaaccagaattccaggttctcctcactgaactccgtcttcaagaaggcacggaatgcagccaccccatacttatgagagagaagcacatcaaaggaatctgcccacctcgtagcttcttctgtcgataatctcttgagagcgcggttgggtttgtctggaagaatagctgtgaaatcactacacgagtctgacttgtgagacaggcatcccagtcgagtcctcatccctttgttctgtctttggccagtcctcatggcctgagggtctttgccaactggatggtcagagaggcttcgggttaaggtgttccacatgggtcttcacactgcctgcttcagttccagaaggaggactctcttcctgcttgccctagtgtagtggttctccaagcgtggtccctgaaccagcagtgtcagcatcacctgcctggcggtgggcagcgcagctgggaaggtgtggctggtgcgggccccagctgggcatggttcggtgaggccctgagtgatagagtcagccacctcctcctggcacctgggagagggtggcagagggcagcccacttcacccagcgcccctagaatagcggctgcaacatgctgctcctgccggctccgctcctctccaggctctgcatctcatgaaaagggaaagagcgagt

SEQ ID NO: 18815 - RNA, 2369 nt, Homo sapiens
  source 1..2369: mol_type = other RNA
tgcaaaagtaatcacagtttttcacactggtccaatggaaatggaagaaacaaacaactccatggatttcactccttctctgagaggtcacctgtcaatgacagaactagaaacctggaattccacagaaacctctctcctaagctgtgagatcccagtgagcagagctggccactacaaatcacagagttgagcccaagtctttcagctattcctcccagggatttacaacaagtggagagtcaggaatcctaaccgaggagggtgtggaggtggtgggaattgcatttgcattatttacagattagcctagcacagcaaatctgccctctcagcagaggtgacccaaggcattatatgaagggcaagttgctgacccagaaaagggtgacagcggcaaggcgctaccactaaccaaaacacaaacatgggtaaatggaatagagtccaagctccggcagctgggtcatactttggaatggcccttcattccctcctcacccccagcctcccacccccaatgccaccgcttttgaacacctatgacatttcacattagaatatgatcttggcagcaagtggaggggaaagccggtgatttccaggagttcccttctgaggtctaactgagcctcctctggctttgggacagcagatctaagtacattttggacctcaggaacctggggtaagagtctttctccatgaggctgtgtacttttccttgggcttggtcaaagcaagtcagggatggctcctgcaggttcttcctcgtggcttctcgggtctggaagtcaatgtttacctcccgtggagcctgcacatccacaaactcctcaaagatcctatgggccttagagaccagttttgcagttgacctggtcttcttgaactcctcacaggccaaccagaattccaggttctcctcactgaactccgtcttcaagaaggcacggaatgcagccaccccatacttatgagagagaagcacatcaaaggaatctgcccacctcgtagcttcttctgtcgataatctcttgagagcgcggttgggtttgtctggaagaatagctgtgaaatcactacacgagtctgacttgtgagacaggcatcccagtcgagtcctcatccctttgttctgtctttggccagtcctcatggcctgagggtctttgccaactggatggtcagagaggcttcgggttaaggtgttccacatgggtcttcacactgcctgcttcagttccagaaggaggactctcttcctgcttgccctagtgtagtggttctccaagcgtggtccctgaaccagcagtgtcagcatcaccttacatcctagcagccacaggagtcggcacatcaaccggtcctgctccagaatggccagtaattcaagacccggccacagacgagacacaggtggttcctgtcaggaacagcatttcctggtatgggaagcctgttctctctggggatgcttggtcagatgggacagtggcagctttgtcttttcattagaaattcctcctgttgtccatctacacaaggggaactgactgtgcagtagaatgactaaagaaagatgctaaagttggaactggggacaatccaagttggcggccactgaatcacgaggagattctatactgccttttgttcttccctccagcttgagtgactcagttgttgaaattttgtggcaagacacctggaagccatttgtcttttttattaaggactcattcacggggtaaaaacgtaataatgttcatttaccatcactccattacccagagcaccagattgctgctaattcaatgtggtgctgattcagtcatcgcatcactgaggcaacattcttctgtgaaagctatttatgtcccggcaccatttgaaaggccctttagatcctttttgaaacattcaagtcccagagaggcagcctgatctgcagagcactgcacaggatgtaggtctgaaaagagccgcttcagagtgacggccagccaacttgaggtcaggccttcaggctcaatgtgcgtccctcttttatcctcaaacgtgcttcagaacgcatcttttcagattcagagagttatggccaacctcagctctgtaaccactccctgcgcactgcaggcaggaagaatttagagggacatgtcagtagctgaacatgtgataacactggctttagactcacccatagcctggcatgagaactcagtcatcctgcacagcttctctgagcccccagtttctccaactcaacaagagggtatttaccccacattgaaacgaggcaagtaaattacaaaaagaggataatgacctagtggtgggtagttggacacccagcagaagccggt

SEQ ID NO: 18816 - RNA, 1648 nt, Homo sapiens
  source 1..1648: mol_type = other RNA
tgcaaaagtaatcacagtttttcacactggtccaatggaaatggaagaaacaaacaactccatggatttcactccttctctgagaggtcacctgtcaatgacagaactagaaacctggaattccacagaaacctctctcctaagctgtgagatcccagtgagcagagctggccactacaaatcacagagttgagcccaagtctttcagctattcctcccagggatttacaacaagtggagagtcaggaatcctaaccgaggagggtgtggaggtggtgggaattgcatttgcattatttacagattagcctagcacagcaaatctgccctctcagcagaggtgacccaaggcattatatgaagggcaagttgctgacccagaaaagggtgacagcggcaaggcgctaccactaaccaaaacacaaacatgggtaaatggaatagagtccaagctccggcagctgggtcatactttggaatggcccttcattccctcctcacccccagcctcccacccccaatgccaccgcttttgaacacctatgacatttcacattagaatatgatcttggcagcaagtggaggggaaagccggtgatttccaggagttcccttctgaggtctaactgagcctcctctggctttgggacagcagatctaagtacattttggacctcaggaacctggggtaagagtctttctccatgaggctgtgtacttttccttgggcttggtcaaagcaagtcagggatggctcctgcaggttcttcctcgtggcttctcgggtctggaagtcaatgtttacctcccgtggagcctgcacatccacaaactcctcaaagatcctatgggccttagagaccagttttgcagttgacctggtcttcttgaactcctcacaggccaaccagaattccaggttctcctcactgaactccgtcttcaagaaggcacggaatgcagccaccccatacttatgagagagaagcacatcaaaggaatctgcccacctcgtagcttcttctgtcgataatctcttgagagcgcggttgggtttgtctggaagaatagctgtgaaatcactacacgagtctgacttgtgagacaggcatcccagtcgagtcctcatccctttgttctgtctttggccagtcctcatggcctgagggtctttgccaactggatggtcagagaggcttcgggttaaggtgttccacatgggtcttcacactgcctgcttcagttccagaaggaggactctcttcctgcttgccctagtgtagtggttctccaagcgtggtccctgaaccagcagtgtcagcatcacctttctcatttccttttgttcctcttgagcattcatttgtctcctcactgctcactgcagggttttcctcttgccagcctcttttctttattcactactttatactcccccttctaagtgtgtcggttggtggtctttctgtaaggagctggcatcatctggtcattgcttgatttgtttcattcagttggtttcttttattgtgtccatcatagtagttaagcaggcaggctctagagccagactgccttggtttaaatcccagctctactattttaaagtgctgtgactttaggcaagtaataaccctgccgtgcctca

SEQ ID NO: 18817 - RNA, 1818 nt, Homo sapiens
  source 1..1818: mol_type = other RNA
tgcaaaagtaatcacagtttttcacactggtccaatggaaatggaagaaacaaacaactccatggatttcactccttctctgagaggtcacctgtcaatgacagaactagaaacctggaattccacagaaacctctctcctaagctgtgagatcccagtgagcagagctggccactacaaatcacagagttgagcccaagtctttcagctattcctcccagggatttacaacaagtggagagtcaggaatcctaaccgaggagggtgtggaggtggtgggaattgcatttgcattatttacagattagcctagcacagcaaatctgccctctcagcagaggtgacccaaggcattatatgaagggcaagttgctgacccagaaaagggtgacagcggcaaggcgctaccactaaccaaaacacaaacatgggtaaatggaatagagtccaagctccggcagctgggtcatactttggaatggcccttcattccctcctcacccccagcctcccacccccaatgccaccgcttttgaacacctatgacatttcacattagaatatgatcttggcagcaagtggaggggaaagccggtgatttccaggagttcccttctgaggtctaactgagcctcctctggctttgggacagcagatctaagtacattttggacctcaggaacctggggtaagagtctttctccatgaggctgtgtacttttccttgggcttggtcaaagcaagtcagggatggctcctgcaggttcttcctcgtggcttctcgggtctggaagtcaatgtttacctcccgtggagcctgcacatccacaaactcctcaaagatcctatgggccttagagaccagttttgcagttgacctggtcttcttgaactcctcacaggccaaccagaattccaggttctcctcactgaactccgtcttcaagaaggcacggaatgcagccaccccatacttatgagagagaagcacatcaaaggaatctgcccacctcgtagcttcttctgtcgataatctcttgagagcgcggttgggtttgtctggaagaatagctgtgaaatcactacacgagtctgacttgtgagacaggcatcccagtcgagtcctcatccctttgttctgtctttggccagtcctcatggcctgagggtctttgccaactggatggtcagagaggcttcgggttaaggtgttccacatgggtcttcacactgcctgcttcagttccagaaggaggactctcttcctgcttgccctagtgtagtggttctccaagcgtggtccctgaaccagcagtgtcagcatcacctttctcatttccttttgttcctcttgagcattcatttgtctcctcactgctcactgcagggttttcctcttgccagcctcttttctttattcactactttatactcccccttctaagtgtgtcttgacctggccatggtgagatgtgggccacactacacactctactgcccactcacttatcacctttccagtctaacacacacttctttcaggaaacctgctctgcctggcggtgggcagcgcagctgggaaggtgtggctggtgcgggccccagctgggcatggttcggtgaggccctgagtgatagagtcagccacctcctcctggcacctgggagagggtggcagagggcagcccacttcacccagcgcccctagaatagcggctgcaacatgctgctcctgccggctccgctcctctccaggctctgggacacaaggaggcgaaacggggtaactggcttgtgggagaaaggataacctgcttt

SEQ ID NO: 18818 - RNA, 1345 nt, Homo sapiens
  source 1..1345: mol_type = other RNA
tgcaaaagtaatcacagtttttcacactggtccaatggaaatggaagaaacaaacaactccatggatttcactccttctctgagaggtcacctgtcaatgacagaactagaaacctggaattccacagaaacctctctcctaagctgtgagatcccagtgagcagagctggccactacaaatcacagagttgagcccaagtctttcagctattcctcccagggatttacaacaagtggagagtcaggaatcctaaccgaggagggtgtggaggtggtgggaattgcatttgcattatttacagattagcctagcacagcaaatctgccctctcagcagaggtgacccaaggcattatatgaagggcaagttgctgacccagaaaagggtgacagcggcaaggcgctaccactaaccaaaacacaaacatgggtaaatggaatagagtccaagctccggcagctgggtcatactttggaatggcccttcattccctcctcacccccagcctcccacccccaatgccaccgcttttgaacacctatgacatttcacattagaatatgatcttggcagcaagtggaggggaaagccggtgatttccaggagttcccttctgaggtctaactgagcctcctctggctttgggacagcagatctaagtacattttggacctcaggaacctggggtaagagtctttctccatgaggctgtgtacttttccttgggcttggtcaaagcaagtcagggatggctcctgcaggttcttcctcgtggcttctcgggtctggaagtcaatgtttacctcccgtggagcctgcacatccacaaactcctcaaagatcctatgggccttagagaccagttttgcagttgacctggtcttcttgaactcctcacaggccaaccagaattccaggttctcctcactgaactccgtcttcaagaaggcacggaatgcagccaccccatacttatgagagagaagcacatcaaaggaatctgcccacctcgtagcttcttctgtcgataatctcttgagagcgcggttgggtttgtctggaagaatagctgtgaaatcactacacgagtctgacttgtgagacaggcatcccagtcgagtcctcatccctttgttctgtctttggccagtcctcatggcctgagggtctttgccaactggatggtcagagaggcttcgggttaaggtgttctcccaccacttgagccaggcagcaagcggccccactgaaagctcttctctctgcttgtcacatccagtaaatactgaagcagcctacacccagcgggcggcggctcagctcccgggcacagtctgcacgcc

SEQ ID NO: 18819 - RNA, 79 nt, Homo sapiens
  source 1..79: mol_type = other RNA
tgcaaaagtaatcacagtttttgccatgagcagtaatggcaaaaaccgcgattacttctcaccaacctgtaacaaaaga

SEQ ID NO: 18820 - RNA, 5695 nt, Homo sapiens
  source 1..5695: mol_type = other RNA
tgcaaaagtaatcacagttttttctctaagaggagaggagttgggacagtggggcaagttggtgagagagcatttctgtgaagagaaacaaagaccaccacgtagtacagccccacatggtgagaagacccgctctcacgggcgggctccgacccctctttaaaaactcttctgcagcagccagactgccaggccagtgcagtcaggaaatggctcaagctcctaaagctagagctttcatttaaaacttcacagcagcccacttagagaaatggcctgtggttcccaccccccaaccccttttctaaggctgctcaagtttgagtttttaaaaagagttcggtagagctaaaggaagctacagtaactcactgcttattaatcaattgcacttaagatctatgttactgattctgaagcgaggcaagcccttgacggaccgcagcctctggccagccagaagtcagggggctcccagacttaggttccacagtggggcccttgtcatcagtggcttttggagctgggactggagcacgtgggtcttttcagaagcccttcttgatgcaaaatttcttatcaatggtatctggagttttgttcatttggcttcaaattgttttttttttttttctaatatattttactgacaagcccttgagagctgctttgctacttgcatgcaggcctctgtgtgaccaggcacacagactacatgtgctccatcttgtctctccgctgctccaggggccttgctcaaaaaccccctatattactggaaactgctggttttacctatgtgcttcttcctaaggcatgcaaaaaaaaatatgtgaaattcagaaaacatttacagttcaggcagctgaggcactgaagtcctaagagacatcacctaaatatcagtggctgtgactcccctgtcccccacaccaattatgaaggtcaggcatgggacacacttgtaattcccctctgctttatggtccagcttaaaacgatgccattagaaggaattctaactcaggtattgcaattatttgaaattcccaatcctcaggagccacacaagcccagggccagcaacaacactttggggagcggggggatgagtttcctgaagtttgtggctgaaaagcaggccttccttggcaaggcttgtgggagcgctgggtgctggagactgaccccacaagtgatcagccaccaggcctaagactaaccagctgcaggacgcccccttccacagtgaggtgaagcctcgccagggggcctgagcagcaggcttgctcttgtccctacattaggacacccgaatggtgtgacaggagagctaaagaaccacccacaaggggaaaagctgatgtcaacttaagagccacacacctctggaaagcaacaagcctctccttcagtttagtccagaagggaaatcccctcatttgtgaacacatcattcatctcaacccaagctgctggctctgtggactgggcctgggcaaggctgtgctgctcctcccaggactgggcccacggccagtacggccagctccttcagggaaacgggcctagcaggggaggcaggcactccactggggaagatggctctcgtggagcagcatctgaggcttgaggcctgtcgtggcctcgcctcccagacacggccacagttcaggcagccagggttccttctaagtcccagtagctcctctgtgtaatcctaatgcttctccccaacctcaagagcccaaaggagatcctgttatcagaaacccagagctcctggactgccagttgcacacgtagacgggcaggccccatctgctcatccttgagtattcccccgacccccaaaatcaatggtgcaggtgatgctcttcagcgctatacagggaataaagacaacatgcactcaagccagcccacacaggccaaggagaacaaagacagccccttaagggagaggcctccagcagagctgaggttaagacacccgttcgtccatctccaaggtggacattctgcaggacgtacgggcccagccttcctctagggcttcagctcaaagaggtcatgatactcctgctgttccagctcctggttatacttctcaatttcccggttggcttcttccacgtagtcattcatgaactggtccatgagtgggtgaaaatcagttttgtcaccaaagaagttaacaaattgggtgccattataaaagtagcctgcaggtaggggttccaagtggcgttttacgtggatgctcctgatctcctgttgcgtcagcatccccctggtcttcagggctttcctctgaggcttctgcttagctgactgccgcagccagtccttgatgctgtcttccttcagggagcagccgatgaacacaaggtagcactcctgctgcccgctgctgtcttgagatacgcttttggagtctggtggtggtgtgggtccttccaaaactggcatgatgctcaaggagttggccagtgtgttgtagcagacctccatggtcctctcagagtctgaaaacttcactttgcccaggatgtggtagatgtttccggagaagggacttggcttgatggaggactgaattgctttacatttggccacaaagcgagtcttctccaagggacggccaaaccatacgcagatctgaaccattaggggatagactgatccagcattcaatttaccttcataccagccaggatacattaaatatcgagatcgtagcatctcaggacttgaaaaactgttttctgagagaatcagctcaatgtcttcattcctggtgacaatcccattttctgcaagaatgaaggctgcagcaggattggcagccctgatgaggctctgcagctgaacaaggagagggtgccgctgctccgtggtgtgactggtgaataccacgttactcaccaggccttgtgaacactggtcaagacatttaggaaagagaaatctgtgctccatgtagcagctcatgggctccacacatgctgtgatggcaccaatggtgaaggaggccttgacatttgagtctgggtgggtctgcagggcctggacaacatcaataacatctgtgtagccttgtaacaccaccagcagtctggtcttcttgcggatgtaggctgactggcgcgcagagcggttctgctgggcctctagggcactggaaaggtatctctggaagtgtgcagcatgaaaacattcagagctgtccatgatttggcgatacaccatccatctgccacattccttatgcagagtgaccagaaaagcacagagctcgctagcgtgacagcctgggaggccggttacaatgctgataattaccttgtcactttctattctgtgagtagtgttgatttcagcttgctgcagcagcacaggaagatgggtccgcatcacaggctcctggctaatgctgctgatggcgaaatgctggagaaaccagtccagctctgggagtttggctgagagtaactttagggaactccgtttctccccagcaggctggctcagggcactgaagagcttctgtgcactggagtgcaatctcttttgttccacagataatccatcttcctggatcacttttaaagagatccctgagttatcctgctgtttccagagggagaagacctctgagtaaaatgcttggtatatcttcgatttggggaaaagggcaatcatcagaaaattgcttgatccatggaaatgaactgggaggtgaggaagcaatgagcttttgaagtctatgagaagagcagcaacagtactggtggaatccccatcatagaaggaaatggaattcatgtgatccttggaaatgatgatacttctatgacgacagtgagaaaacagaaggccactagagaagaaatgaacattcccttcctcaggccaggactgtagattgctggaataaagatatgctccttctcctcctgttagataagtgcccaggaaagactcatcccccctcactgcttgctgggttttctcagacaattttacttcattatcttccaccagccaggagcagaatctgggtacagcagcagtcaggactacggagctggtttctgtggtaacagtgccatccttttctttaactaagatctgagaagtcaaaaatgattcagagaaaaccacagatcctaaacaaccattgcctcccagtaagtcaggaatgtcatagacggccatacaagccgtcttcacaaaggataagctatcttcactgtccagcggtacaattcttccctgattattcacagcatgtatatgaaaagtcatcttggagcgcagggctgccttaaacggaatcaactcaaaggaatctaacccagatcccagagtttgctctgctacctccttggcctttgttagactggaagttttagcataacatgcaatgccagccaaaacagcctcaataacagcagcatatatctgggacaatagcctaatttgttcagttttcttgggcagcttgctgtcaccacccaagtaaggaacatgagtagctccaaaaaagtatgttctcgaacaagcaagaggtccctttggtgagacacactgggctaccatgtgcttggcaaagctcccgccgggaccagtgcttcgtaccagatgtccttcagaagggaagttaaagttgccagcattcaggttttctcgtgtggagtgattaccaaagagaacaaatggctgccggttagggctgttttcagttatatggctagagatcattccatgactgaaataacttctgaatggctcacccgcctgagattctgaaagttctagcaggaaaggaatttctgtgtcaaaattagcgaagaagctagtccactgatgttcaaaagccaccaaatcatctgaaagcaaactctccagagacataggatccatcttgctgtagacattccatagattcaaactcacatcctgcaactcatatttcatggtaaaaaatccatcccctccaatgccctcaagtgcaaaggcctgtacaattggccatttctccaccacaaacatatcaaatatctgcaagtgaccttgggagctgtaaggaatgccaattctactacagtctcgaaccatgtccacaaagctggtaattttaaattcttctgcggcttcttcatcttcatactcattttcggtcatgcagtggaaatgcagatttctccaatgtgccacataaggtaagagatagcgaaagtttacaggattacagtacagatggacgctatccgatttaatcaatataattacatcatctagtacttcttcagaaaatcccgttttctcaaaatcactggtattctgattgtacaaaccaaatagaagataatttgccagctctctgcagccttcattgtacctgctatcgattcctaggatgcagaggatcccatccggccgagacttgctgctctgggtcaggatgctctgaacctgccgaagtcgactgcagctgacggagggtgacccgcggctggagccgccaggggaccgagcgcggggcagcccctgccggcgcggggggtacacgtccatggcggcggacgactggcggcggaggaggacggtgcagctgcgagggtctcagttgcccgcagggcggctccacgctagctgcggccgggcggggcggcagggcgtgccgggt

SEQ ID NO: 18821 - RNA, 5597 nt, Homo sapiens
  source 1..5597: mol_type = other RNA
tgcaaaagtaatcacagttttttctctaagaggagaggagttgggacagtggggcaagttggtgagagagcatttctgtgaagagaaacaaagaccaccacgtagtacagccccacatggtgagaagacccgctctcacgggcgggctccgacccctctttaaaaactcttctgcagcagccagactgccaggccagtgcagtcaggaaatggctcaagctcctaaagctagagctttcatttaaaacttcacagcagcccacttagagaaatggcctgtggttcccaccccccaaccccttttctaaggctgctcaagtttgagtttttaaaaagagttcggtagagctaaaggaagctacagtaactcactgcttattaatcaattgcacttaagatctatgttactgattctgaagcgaggcaagcccttgacggaccgcagcctctggccagccagaagtcagggggctcccagacttaggttccacagtggggcccttgtcatcagtggcttttggagctgggactggagcacgtgggtcttttcagaagcccttcttgatgcaaaatttcttatcaatggtatctggagttttgttcatttggcttcaaattgttttttttttttttctaatatattttactgacaagcccttgagagctgctttgctacttgcatgcaggcctctgtgtgaccaggcacacagactacatgtgctccatcttgtctctccgctgctccaggggccttgctcaaaaaccccctatattactggaaactgctggttttacctatgtgcttcttcctaaggcatgcaaaaaaaaatatgtgaaattcagaaaacatttacagttcaggcagctgaggcactgaagtcctaagagacatcacctaaatatcagtggctgtgactcccctgtcccccacaccaattatgaaggtcaggcatgggacacacttgtaattcccctctgctttatggtccagcttaaaacgatgccattagaaggaattctaactcaggtattgcaattatttgaaattcccaatcctcaggagccacacaagcccagggccagcaacaacactttggggagcggggggatgagtttcctgaagtttgtggctgaaaagcaggccttccttggcaaggcttgtgggagcgctgggtgctggagactgaccccacaagtgatcagccaccaggcctaagactaaccagctgcaggacgcccccttccacagtgaggtgaagcctcgccagggggcctgagcagcaggcttgctcttgtccctacattaggacacccgaatggtgtgacaggagagctaaagaaccacccacaaggggaaaagctgatgtcaacttaagagccacacacctctggaaagcaacaagcctctccttcagtttagtccagaagggaaatcccctcatttgtgaacacatcattcatctcaacccaagctgctggctctgtggactgggcctgggcaaggctgtgctgctcctcccaggactgggcccacggccagtacggccagctccttcagggaaacgggcctagcaggggaggcaggcactccactggggaagatggctctcgtggagcagcatctgaggcttgaggcctgtcgtggcctcgcctcccagacacggccacagttcaggcagccagggttccttctaagtcccagtagctcctctgtgtaatcctaatgcttctccccaacctcaagagcccaaaggagatcctgttatcagaaacccagagctcctggactgccagttgcacacgtagacgggcaggccccatctgctcatccttgagtattcccccgacccccaaaatcaatggtgcaggtgatgctcttcagcgctatacagggaataaagacaacatgcactcaagccagcccacacaggccaaggagaacaaagacagccccttaagggagaggcctccagcagagctgaggttaagacacccgttcgtccatctccaaggtggacattctgcaggacgtacgggcccagccttcctctagggcttcagctcaaagaggtcatgatactcctgctgttccagctcctggttatacttctcaatttcccggttggcttcttccacgtagtcattcatgaactggtccatgagtgggtgaaaatcagttttgtcaccaaagaagttaacaaattgggtgccattataaaagtagcctgcaggtaggggttccaagtggcgttttacgtggatgctcctgatctcctgttgcgtcagcatccccctggtcttcagggctttcctctgaggcttctgcttagctgactgccgcagccagtccttgatgctgtcttccttcagggagcagccgatgaacacaaggtagcactcctgctgcccgctgctgtcttgagatacgcttttggagtctggtggtggtgtgggtccttccaaaactggcatgatgctcaaggagttggccagtgtgttgtagcagacctccatggtcctctcagagtctgaaaacttcactttgcccaggatgtggtagatgtttccggagaagggacttggcttgatggaggactgaattgctttacatttggccacaaagcgagtcttctccaagggacggccaaaccatacgcagatctgaaccattaggggatagactgatccagcattcaatttaccttcataccagccaggatacattaaatatcgagatcgtagcatctcaggacttgaaaaactgttttctgagagaatcagctcaatgtcttcattcctggtgacaatcccattttctgcaagaatgaaggctgcagcaggattggcagccctgatgaggctctgcagctgaacaaggagagggtgccgctgctccgtggtgtgactggtgaataccacgttactcaccaggccttgtgaacactggtcaagacatttaggaaagagaaatctgtgctccatgtagcagctcatgggctccacacatgctgtgatggcaccaatggtgaaggaggccttgacatttgagtctgggtgggtctgcagggcctggacaacatcaataacatctgtgtagccttgtaacaccaccagcagtctggtcttcttgcggatgtaggctgactggcgcgcagagcggttctgctgggcctctagggcactggaaaggtatctctggaagtgtgcagcatgaaaacattcagagctgtccatgatttggcgatacaccatccatcttgtcactttctattctgtgagtagtgttgatttcagcttgctgcagcagcacaggaagatgggtccgcatcacaggctcctggctaatgctgctgatggcgaaatgctggagaaaccagtccagctctgggagtttggctgagagtaactttagggaactccgtttctccccagcaggctggctcagggcactgaagagcttctgtgcactggagtgcaatctcttttgttccacagataatccatcttcctggatcacttttaaagagatccctgagttatcctgctgtttccagagggagaagacctctgagtaaaatgcttggtatatcttcgatttggggaaaagggcaatcatcagaaaattgcttgatccatggaaatgaactgggaggtgaggaagcaatgagcttttgaagtctatgagaagagcagcaacagtactggtggaatccccatcatagaaggaaatggaattcatgtgatccttggaaatgatgatacttctatgacgacagtgagaaaacagaaggccactagagaagaaatgaacattcccttcctcaggccaggactgtagattgctggaataaagatatgctccttctcctcctgttagataagtgcccaggaaagactcatcccccctcactgcttgctgggttttctcagacaattttacttcattatcttccaccagccaggagcagaatctgggtacagcagcagtcaggactacggagctggtttctgtggtaacagtgccatccttttctttaactaagatctgagaagtcaaaaatgattcagagaaaaccacagatcctaaacaaccattgcctcccagtaagtcaggaatgtcatagacggccatacaagccgtcttcacaaaggataagctatcttcactgtccagcggtacaattcttccctgattattcacagcatgtatatgaaaagtcatcttggagcgcagggctgccttaaacggaatcaactcaaaggaatctaacccagatcccagagtttgctctgctacctccttggcctttgttagactggaagttttagcataacatgcaatgccagccaaaacagcctcaataacagcagcatatatctgggacaatagcctaatttgttcagttttcttgggcagcttgctgtcaccacccaagtaaggaacatgagtagctccaaaaaagtatgttctcgaacaagcaagaggtccctttggtgagacacactgggctaccatgtgcttggcaaagctcccgccgggaccagtgcttcgtaccagatgtccttcagaagggaagttaaagttgccagcattcaggttttctcgtgtggagtgattaccaaagagaacaaatggctgccggttagggctgttttcagttatatggctagagatcattccatgactgaaataacttctgaatggctcacccgcctgagattctgaaagttctagcaggaaaggaatttctgtgtcaaaattagcgaagaagctagtccactgatgttcaaaagccaccaaatcatctgaaagcaaactctccagagacataggatccatcttgctgtagacattccatagattcaaactcacatcctgcaactcatatttcatggtaaaaaatccatcccctccaatgccctcaagtgcaaaggcctgtacaattggccatttctccaccacaaacatatcaaatatctgcaagtgaccttgggagctgtaaggaatgccaattctactacagtctcgaaccatgtccacaaagctggtaattttaaattcttctgcggcttcttcatcttcatactcattttcggtcatgcagtggaaatgcagatttctccaatgtgccacataaggtaagagatagcgaaagtttacaggattacagtacagatggacgctatccgatttaatcaatataattacatcatctagtacttcttcagaaaatcccgttttctcaaaatcactggtattctgattgtacaaaccaaatagaagataatttgccagctctctgcagccttcattgtacctgctatcgattcctaggatgcagaggatcccatccggccgagacttgctgctctgggtcaggatgctctgaacctgccgaagtcgactgcagctgacggagggtgacccgcggctggagccgccaggggaccgagcgcggggcagcccctgccggcgcggggggtacacgtccatggcggcggacgactggcggcggaggaggacggtgcagctgcgagggtctcagttgcccgcagggcggctccacgctagctgcggccgggcggggcggcagggc

SEQ ID NO: 18822 - RNA, 5205 nt, Homo sapiens
  source 1..5205: mol_type = other RNA
tgcaaaagtaattgcagtttttgaggcgtacaagtcagttattttgttaaaatctccctcaatatgggtttgtctgatgttttctgatttagattacatatttttgccaagaataccacaaaagtgacgttgtgctctcatgagcacatcctgtaaaaaaggtatataatgtagattcgtcccaatactgattcaatcacttgggtaagatggtatctacccggtttctccactgtgatggagattacagtgcagagtggaaattttcttgctattacagaacctcatgatttctacagcttatggtttttgcgatcagtatttcgttggtttgaaagaactctgctaaagaaaaagagaacccaacatttgcccagaagactagagactgtgtttaccggaagtgtgcttttctaaaaaaaagtttaagcctcctccccgtcggggaatcgaaccccggtctcccgcgtgacaggcggggatactcaccactatactaacgaggaattgacgtgaaaatggagctcttaggaaatccctgtgaagttactcgctattgtccatctttctttgctctgtagtcacacgtttcccctaccaaatatacgcaaggcaattcagcgaacgtgtctccgcccaaccgcgaatcctctccagttcctccttcattcctcggacgctttgtcagacccttttaaaaaagaactctcgctagcctcctttgtgacgcactggtttccgtctatgttcaaccatggttggagccctagctaacataggagttacaaatcccgaaaggtgcatcggttggtttcaaagacaggaaaagcagaggtgggaccaatacctgcgctccgttgaggtaaaatagataaagagtctgcagatgtatttttaaagttcaggatgcgtcaagtggcacgcagaagctttatcacgagttccctcgcccccaaactgaaagcaaatatgacatcgtatttcctctctgaagtaaatacgattcctctctgttctcagtaaaacatcccgaagtcggcaaaagttcaggctgcgttaagtggcacgcagaagctctattacgagttcctttactcccaaactgaaagcaaatatgacatcgtatttcctctctgaactgttctcagtaaaacatcccgaagtcggcaaaagttcaggctatgttaggtgacacgcagaggctctatcacgagtttctttactcccaaactgaaagcaaatgtgagatcctatttcctcgctgaactgttctcagtaaaacatcccgtagtcggcaggattcgaacctgcgcggggagaccccaatggatttctagtccatcgccttaaccactcggccacgactacacgaatggagaaggctcccttcacatctttaaacagaatttacaccagctaactgacaagaaacggtcaaaagaacaaaatacggtaaaaatggtttcctgggcaagaaactggagtctgcgagttcattagaaactctaacgtgaagtgcaagttggataagacaagccaacctctctggggcagccgcaaggagtccttgccctatcagcagtaccgtttccagaaaactagagaccactgtacctctctcacctggacccaaactgaccccgcaaggaagtggaatcagaccctcaccgtaaatctgggcctgacacatttagtttttgtttgaaacttcctctcattgaggctccttgatgaatgctaatggctttcaagaagggactaacttttgatttgtgtctgaactggagggccagaaaatgatgcagaaaagcctacttgcactttcttgctctgatgaggtccctaagtctctaggctcacaccaacccaagggagtatatctacccggtctcgtttgcacggcattttgcatttcacaatgcgcttccacgcttcagttgggttaagaaagaaatttatagattgttcatgagttcccatggaaccaggttacctatcaaaaggaagatcctactttgatttttggccaaggcagacgctccttctctcaaaatctaacccacgcagtatgttttcttttcctcttatgcttccgtcttgaagtctaaagctgccggtcctggagtttccctgagccctttggatgcacagattattgtaattggctttcatctacttcttggaaccatatactaatctaagaaaagagggaaacaatcgcaagctaagaaatcatgtcgactaagtagataaatgaggaagagggacaagaaggaagaggaaaagaagaaagtgaccagaaaggagaagagagaaaggaaggagggacaggaggtagaaagaagaggatgaaggagaaagaagaggaggaagaggaagaggagaaacgaaggaagaccgggaagggaagagacagagattttctgaggacccttgttagagctcagaaaatgataccccaaagtatggctcttggaagtgctgagtactttgaactaaagaagcaacctcagaatcaaagtctctctgaccttccgcagccccactgcctcctgatcctctttctttcttgaatggcagggaggggctttcactgaagtttcccttatttgacttacggaggttcctccagaaggaaagagattgtcatgaaccctctcctggaatctgtattaaccagagaagattaactcagatcccaggagagaaaactaaaggtctccatgcccgggacatctcgcccagccagacttcaattcttttcttcaccacctattctgagggctgctacttgagagactttatctgtataataagacaagctttgttcccagagctgttcctgccctgaccctcacattgcttctcgccaccaccttccaggagccttcaagctcctatttctttatgtagctccaagtcctatttaagcttcaaccatctgccccttctttgagtctcacttacactttctgggacctctgtgcatatgtgcataataaatgtgtatgccttttcttctgttaatctgtctactagcagctttatttctcagactcaaatatccaacctccagaagggagaaaaaagattctctcacccctacaggctcaaaagaagactaaaagaaattcactagttttatggaagaccataatttgagggaatagacatgaagcagtttgatggggtagccaggtgtccatacaaatataagttgtgctatagattgttgttcatagttaatgcatatcacatcctttttatttggtggacatatttttatcaagcacatctttatttttttttgctgaaatcatttgcaactccagctttgaataaagttagataccaaagaaatatcaaatctcttttaagaaatttaaaaaaattttagaatcagggtcttactctatcacacagactggagtgcagtggcaccatcatagcttactgtaacctgaactcttgggcacaagccatccttctgcctcagcctccagagtagctaggaatagaagcatgcaccaccactcctagctaacttttttttctttgtagaaaaaaaatgtattttctttgtattccttgtatttgaagaaaaactgacaatttgcctttttaagtatagaaggacatttgatttgtttccaatttagggctaaagtagaaactggactggtttttgtttcctgcaactaagtcctgactctctacctttactgagatccattctactatgtttttgttttcagcccagtaaaacaagtaagattgcagctgtggccagtccctagtcattgttacagtaaaacaagccaaagttgattagtaatttcagttcaaatatatcactagttgctttgtattttgctgaggtgtttttttaagcacaaaaggtttctgagggctgggttcagtggcttatggactgtaaccccagcatttaggaaggccgaggtgggaggattgcttgaggtcaggagttggaggccactttgtgcaacatatagagaagtcactgaagacaaaaattatatctttctgtgtcctcaacatgtattgaaagcctcatttgtataaggtatggctaaaagttttccaaatcatgagtgctggttcctttgtgctgaatagttccttcctcagtttatttctttcctcatgcatttcaccataagcagcaataactaaccaggttgcacattccacattttacttggaagtcttcttaactaaatattcaagttcatcatgtacaaattctgttttccacccaaatatagaatacaattcagccaaggctctcccactttataacaagataaccattccttcagtttctaattgcatgtcattaatttccttctgagaccttaccataagcatatttaacattcttatattttaaatttaatagaacattttgggaacagttttaggtttatagaaaaattgagcagaaagtagagtttcagtatactccttccttctcccctcctcccccagtttctctattattaacatcttgcactagtgtggtacatctgttaaaattgatgagccaatgttgataaattattattaactaaagaccatagtttatattacggttcactctttgtgctgtatattctatgggttttaacaaatgtataacaacatgtattcgccattacaatatcatacagaatagtttcactgccttaaaaatccactgaacgtcacttattcttccctcttaaaatccactgaacgtcacttattcttccctcttaaaatccactgaatgtcacttattcttccctttttccctccccctaagcccctggcaaccaccaatctttgctgtttccatagattagccttttcaggaatgttatgtagatggaattatacagtatatagccttttccagattgacttctttcactcaccaatacgcacttaatattcttctgttcttcctttttggtagcttgatagctcatttcttttccttactgaatgttccattgtctgaatgtaccatagtttatgtattcattcatgtactgaaggacatctggctgcttccaagttttgcctgaaacaggagcaaaagactggcggcgaaaatgtgcggcccatcgcagggcgaaagtacacgttagctaaagcctctgggaaatgaagttcaggaacaccttcgcggagtgttctggg

SEQ ID NO: 18823 - RNA, 519 nt, Homo sapiens
  source 1..519: mol_type = other RNA
tgcaaaagtaattgcagtttttgattccacaaccctgtataacttggcattctggtgaattggacccgaacatctgtgaatcttaaaaatagtggttgactcattatggcttccttatgtataggattaagaacacagatcctggaatcagacagcctggcttccacactctagctgggtgaccatgaccatgaagaagttcctgaatgttccagtgtcagtttattcacctttacagagaaatctggcaaacactacctcagccaggtgatcaagttcaatattcagcaataagtcatgttgtttgttagtgtgtgctcttgatatgacatgatgagaattgcacttcacttctgtgatattccccatggggttggaagaacaaaggaagaaaacagtgtctctgctgcagtagaggaaggaccacaggtagaggtcggtagaggtcagcaatggaagcgctgggttgctgccagtgagagaggcaaaactcggagggggcaggaaggaagttcccta

SEQ ID NO: 18824 - RNA, 720 nt, Homo sapiens
  source 1..720: mol_type = other RNA
tgcaaaagtaattgcagtttttgattccacaaccctgtataacttggcattctggtgaattggacccgaacatctgtgaatcttaaaaatagtggttgactcattatggcttccttatgtataggattaagaacacagatcctggaatcagacagcctggcttccacactctagctgggtgaccatgaccatgaagaagttcctgaatgttccagtgtcagtttattcacctttacagagaaatctggcaaacactacctcagccaggtgatcaagttcaatattcagcaataagtcatgttgtttgttagtgtgtgctcttgatatgacatgatgagaattgcacttcacttctgtgatattccccctggctttaacttcagatcactgaaagaaacactgaagaggtaggaaaagaagtcttgaatcactgatgccacctctcctgcaatccttggccgcagtggagagtgtttctgtgccaaagctcttagacaacaccagcggccagaacccaccccagccagttgcaataatctctgggaatgccagcccaggcaccggtagttttcaaaagctcccttggtggtcacgtgcagcaagggttgagaaccactgatgtaagttaatagtctttagtgaagggcctacttacagagatttgggcagcattaaggaaccaaaaaatggcatgttgaagcacccaggtaccagcaagag

SEQ ID NO: 18825 - RNA, 635 nt, Homo sapiens
  source 1..635: mol_type = other RNA
tgcaaaagtaattgcagtttttgattccacaaccctgtataacttggcattctggtgaattggacccgaacatctgtgaatcttaaaaatagtggttgactcattatggcttccttatgtataggattaagaacacagatcctggaatcagacagcctggcttccacactctagctgggtgaccatgaccatgaagaagttcctgaatgttccagtgtcagtttattcacctttacagagaaatctggcaaacactacctcagccaggtgatcaagttcaatattcagcaataagtcatgttgtttgttagtgtgtgctcttgatatgacatgatgagaattgcacttcacttctgtgatattccccctggctttaacttcagatcactgaaagaaacactgaagaggtaggaaaagaagtcttgaatcactgatgccacctctcctgcaatccttggccgcagtggagagtgtttctgtgccatggggttggaagaacaaaggaagaaaacagtgtctctgctgcagtagaggaaggaccacaggtagaggtcggtagaggtcagcaatggaagcgctgggttgctgccagtgagagaggcaaaactcggagggggcaggaaggaagttcccta

SEQ ID NO: 18826 - RNA, 3702 nt, Homo sapiens
  source 1..3702: mol_type = other RNA
tgcaaaagtaattgcagtttttgccactgaaagtaatggcaaaaaaaaaaaaaaaaggaagtactggctattatcagatgtgtaattagttgtgtccttctccaccagagggcgcagtcctgcacccgagacttgtcacgaaaacccgataatggggtagatctgaaagtaggttcatgaccccagtcattgataacagcagtcactggtggaatcaggggactctgcagtcacaggactcaaacttggaaatgagacatcatctagaaacctagatgatcacagggcctcaaattgtagtattcaagttcccctttcatgtacatattcagcattttccaagccttcagacaagatttctcccttttggtttgtctccccatggggacaaatgtattctaatttatttttactctggtaaattataaagtaatgaatgacagatagttctaacttaattgacgggctccccaccatattgcaaataaaatgacttgaaaattgtcatctcagaagcctatgtctgcatttaatttttgtaatctaggactcttttccacctaaagccaataaataaggaaactgtatttccacttctttccactgtactttggcaaaaatagattctggacttcttactactatttcattgtgccctttcaggtggatgtgagtctgtgtcatttattggttacatccttacacatgtatcattcttacccatctcttagtcccgtctaccatggaaacagtaggtgatgacaggatggtaataagcatgaaattcaaaaccagaaaggtgagctgatgctggagctacagggtctttactatctgcaactggagtggaccatttctgctgtcttgtccttgatatgacactgacatgaagatacagtaagaacatttgccatttctggtgctcttcattcctttgggcaaattcaagtgtccatctggtataattttccatcagtttgaacaacttcctttagcatttctcgtagtacagttttagtgatgaattctttcatctttagatttcctcagaaagaaatgatggtattgcggtgcctcagctctaccaactagattcaccaaccagtgagctctgcctcaatcatcgtagaatcaggaatcatcatctcggagtcattctgagatgattcatcatagaattgggaatcatctcagagtcattatcagagtctcagatcatcagtattataatccctattgcacttttcttgaagcattttaccttcctgaccggacaccatctgttcctgtgagtagaaaaatcctacggtctctgcaattctccttctgtgaagaggcctggatggaggcagcttcctgcagcctctcagggtggcagggatctcctagcaggttgattgtgtcacgggatccttcaggtgttgcttttccagctagaaagctctgtgaccagtggtgcctttgcctgagttttgatcaggcccgccagacttgttccactgacgtggcctggcaggctgtgctcagctcatgctaccagccaggattccacgcctgccgagggtgagccaggcacggaacagcgaggggtgtgcaggcgagcgaacgcagggtctggccactgcgcagagccggacacaccagctgctgcagctgggcaggcagctccaggcgccggcaaaggtgccggttctatgcaagtctgcagctggatctgatgaaccacaagcggcttctgctgtgggcacctgtgtctggacaaggggaatgcagtggtgcccggaagtttgaagataccagaaaccgcagagccccaaagagggtgtcacagccctggctcagggagcccctaggtctgtgctccctgaagggccacagcacttctctccttcacatcacccgcaacatggcaagtcgcgggggtgtggggacgggaggagggcgtgtttcagccctgtttgtgttactgctctttcagtcccgccattcagtgggtcctgagttctcgtcccacatccaggaagaatgaggtacgcggacaactagagggtgagcaaggcggagaggagccttatcgagtgacagaacagctctcgggaaacttgaagtgggtagctcctttccgcaggcaggttgtcccagtaagtgtccagctctcagtggagaagagacccagagtgggtagctcccttcttcaggcaggttgtcttgatgagtcgaggagacctgaattgggtagctccttcccacagctggtagtcccagcgtctgtgtgagtctggctaggctcagaagggaggaagtgcatgctgattggcccatgggtggccatgggctgacccggaaaaatcaccataagttctcactccgggccacagacttcacccgggactgacagcctagcccctgggcttcaggcctccctggcttgatggtggggctttaccggggacccacctctttccgcccaggagcctgtctgcctcctgccaccatcaatcatgtcatccacagcgcccaggctgttcctgcagaggagtaccggcagcccgcaccgagtgccctcagctcccccaccccacgccgccagcctctctcctgtgcttctcagtgcccaaagcctagagggggccagggtggcagggggctggcatgtcagcggcgccccaggcgcacgcacacccagctgggtctagacagcgcttggcctcagccacaactttgctccaccccagagtgggctccaggagcaaggagaggccaggcagcaggagcaggcacttccaagcctgcgggtcagggggtcttcccagcccccgagagcacagggatgtccaggtctgcagctgtggctgggtggttgcagctgtgccggaaagcgtggggctcccacccggccaactcagaagagggtggggctccggccagctccacggagcacgcagcccccaccgtgcctcccacactacagctggcatcttcacagtagccgctccagacaggccactgctgccatcaattgtttacttgtcttaaactgcaggtgttcataacccatattgcagagctctacttatcagtcctattcttgtgattggggacagggatgcaaagcagaggagaaaggcttacgaagaggaagaggttgaggagactggaactgtcaagagcactcccccaacatcctccaccttcagaatgagttttcaggtaataacttctgttgttgccagcagactatgccaaacattcacttgcaccagggccagaacattggtctgttccttgttcctcaggccagaggctgtttgggtgcagggtactctcgcgtttccttctttgaagcatcctctattttcctggattcacttaggaaattctaaaagaatatacgagctcacattcctttggtcataagagcagtgtcatcattagacatcaggtcgcctctggaaaattccattgtgagtttaaaaggcaaatgacgtctataattctaaaactagttctcccaccgaaactctagaaaggatcttgggatctgcagggtctcccggatcacactttgagaactgctgctttagtcttcctcccatctcctaaggccagagctcctgagtttgcttcccactggccaaggagaaaagagcaaggtcacttgtcggggggctgcagagggaattaccttctttcatttgcaaa

SEQ ID NO: 18827 - RNA, 3706 nt, Homo sapiens
  source 1..3706: mol_type = other RNA
tgcaaaagtaattgcagtttttgccactgaaagtaatggcaaaaaaaaaaaaaaaaggaagtactggctattatcagatgtgtaattagttgtgtccttctccaccagagggcgcagtcctgcacccgagacttgtcacgaaaacccgataatggggtagatctgaaagtaggttcatgaccccagtcattgataacagcagtcactggtggaatcaggggactctgcagtcacaggactcaaacttggaaatgagacatcatctagaaacctagatgatcacagggcctcaaattgtagtattcaagttcccctttcatgtacatattcagcattttccaagccttcagacaagatttctcccttttggtttgtctccccatggggacaaatgtattctaatttatttttactctggtaaattataaagtaatgaatgacagatagttctaacttaattgacgggctccccaccatattgcaaataaaatgacttgaaaattgtcatctcagaagcctatgtctgcatttaatttttgtaatctaggactcttttccacctaaagccaataaataaggaaactgtatttccacttctttccactgtactttggcaaaaatagattctggacttcttactactatttcattgtgccctttcaggtggatgtgagtctgtgtcatttattggttacatccttacacatgtatcattcttacccatctcttagtcccgtctaccatggaaacagtaggtgatgacaggatggtaataagcatgaaattcaaaaccagaaaggtgagctgatgctggagctacagggtctttactatctgcaactggagtggaccatttctgctgtcttgtccttgatatgacactgacatgaagatacagtaagaccacacatttgccatttctggtgctcttcattcctttgggcaaattcaagtgtccatctggtataattttccatcagtttgaacaacttcctttagcatttctcgtagtacagttttagtgatgaattctttcatctttagatttcctcagaaagaaatgatggtattgcggtgcctcagctctaccaactagattcaccaaccagtgagctctgcctcaatcatcgtagaatcaggaatcatcatctcggagtcattctgagatgattcatcatagaattgggaatcatctcagagtcattatcagagtctcagatcatcagtattataatccctattgcacttttcttgaagcattttaccttcctgaccggacaccatctgttcctgtgagtagaaaaatcctacggtctctgcaattctccttctgtgaagaggcctggatggaggcagcttcctgcagcctctcagggtggcagggatctcctagcaggttgattgtgtcacgggatccttcaggtgttgcttttccagctagaaagctctgtgaccagtggtgcctttgcctgagttttgatcaggcccgccagacttgttccactgacgtggcctggcaggctgtgctcagctcatgctaccagccaggattccacgcctgccgagggtgagccaggcacggaacagcgaggggtgtgcaggcgagcgaacgcagggtctggccactgcgcagagccggacacaccagctgctgcagctgggcaggcagctccaggcgccggcaaaggtgccggttctatgcaagtctgcagctggatctgatgaaccacaagcggcttctgctgtgggcacctgtgtctggacaaggggaatgcagtggtgcccggaagtttgaagataccagaaaccgcagagccccaaagagggtgtcacagccctggctcagggagcccctaggtctgtgctccctgaagggccacagcacttctctccttcacatcacccgcaacatggcaagtcgcgggggtgtggggacgggaggagggcgtgtttcagccctgtttgtgttactgctctttcagtcccgccattcagtgggtcctgagttctcgtcccacatccaggaagaatgaggtacgcggacaactagagggtgagcaaggcggagaggagccttatcgagtgacagaacagctctcgggaaacttgaagtgggtagctcctttccgcaggcaggttgtcccagtaagtgtccagctctcagtggagaagagacccagagtgggtagctcccttcttcaggcaggttgtcttgatgagtcgaggagacctgaattgggtagctccttcccacagctggtagtcccagcgtctgtgtgagtctggctaggctcagaagggaggaagtgcatgctgattggcccatgggtggccatgggctgacccggaaaaatcaccataagttctcactccgggccacagacttcacccgggactgacagcctagcccctgggcttcaggcctccctggcttgatggtggggctttaccggggacccacctctttccgcccaggagcctgtctgcctcctgccaccatcaatcatgtcatccacagcgcccaggctgttcctgcagaggagtaccggcagcccgcaccgagtgccctcagctcccccaccccacgccgccagcctctctcctgtgcttctcagtgcccaaagcctagagggggccagggtggcagggggctggcatgtcagcggcgccccaggcgcacgcacacccagctgggtctagacagcgcttggcctcagccacaactttgctccaccccagagtgggctccaggagcaaggagaggccaggcagcaggagcaggcacttccaagcctgcgggtcagggggtcttcccagcccccgagagcacagggatgtccaggtctgcagctgtggctgggtggttgcagctgtgccggaaagcgtggggctcccacccggccaactcagaagagggtggggctccggccagctccacggagcacgcagcccccaccgtgcctcccacactacagctggcatcttcacagtagccgctccagacaggccactgctgccatcaattgtttacttgtcttaaactgcaggtgttcataacccatattgcagagctctacttatcagtcctattcttgtgattggggacagggatgcaaagcagaggagaaaggcttacgaagaggaagaggttgaggagactggaactgtcaagagcactcccccaacatcctccaccttcagaatgagttttcaggtaataacttctgttgttgccagcagactatgccaaacattcacttgcaccagggccagaacattggtctgttccttgttcctcaggccagaggctgtttgggtgcagggtactctcgcgtttccttctttgaagcatcctctattttcctggattcacttaggaaattctaaaagaatatacgagctcacattcctttggtcataagagcagtgtcatcattagacatcaggtcgcctctggaaaattccattgtgagtttaaaaggcaaatgacgtctataattctaaaactagttctcccaccgaaactctagaaaggatcttgggatctgcagggtctcccggatcacactttgagaactgctgctttagtcttcctcccatctcctaaggccagagctcctgagtttgcttcccactggccaaggagaaaagagcaaggtcacttgtcggggggctgcagagggaattaccttctttcatttgcaaa

SEQ ID NO: 18828 - RNA, 59 nt, Homo sapiens
  source 1..59: mol_type = other RNA
tgcaaaagtaattgcagtttttgccactgaaagtaatggcaaaaacagcaattactttc

SEQ ID NO: 18829 - RNA, 60 nt, Homo sapiens
  source 1..60: mol_type = other RNA
tgcaaaagtaattgcagtttttgccattactttctaatagcaaaaatcacagttaccttt

SEQ ID NO: 18830 - RNA, 65 nt, Homo sapiens
  source 1..65: mol_type = other RNA
tgcaaaagtaattgcagtttttgccattacttttaaatgacaaaaaccacaattacttttgcaca

SEQ ID NO: 18831 - RNA, 4378 nt, Homo sapiens
  source 1..4378: mol_type = other RNA
tgcaaaagtaattgcagtttttgccattacttttagtagcaaaaaccacaattacttttctatcaatgtaatagtagaaacggggtttcactgtgttggccaggctgttcttgaactcctgacctcaagtgatccgcctgcctcagcctcccaaagagctgggattagaagtgtgagtcactgatcctggctgaaataaaaaaaattaaaaaatatattttattgttttgaattttatttaaaactctttgcaagaaatgatgctggaagactacctgtttagaattgtaatccatatatccacaagctctggcagctttaaagagaggcaatagaagaatgaatgcccaaatgtagcagattggcttttactcattttcatagtctcctcaccctagcactggtataatatgattctgagaatgttaggcagctaaagctgtttcttttaattcttgtccactttggtgacatgaggaatcaaactcaccattttatatatttagatactgaatattctggtagctcagcaccagactctgtgaagtcattccttttgcttatctatgacttggattacattccaagtatgaattaacatacagccagactagatgaacagctttagaagaatatgacttgcttttttttttttgacaagctcatttagaaggtgatacattcttttccatgttcatttccaaatgcttatataaagaatgctgagtgaactcttgcctagtgatcttaaacattaacttacacaaagtaccttccttccttgtctcagcatgttaatacatcctgtctctcccatagatatctagggcaatgaagttgatgctagcccagttcttataacctgctgccaagtattttgatggctttatctgaagagtaggtaagatctttgctgacccagctacccagcatgcagctggatgtgtggagagtagaaatatgctggccttgtgcagatggatttcaagtacaatggccaacatttttactgtccctgctatattaaaccaaccaatttaatgccttctttctagttaagctccagttccttgaaaaatatattgtttataatatagttataatagatgtcatttattaaacacaataaatactggctgtcttttaatattttacatctattttctcagtgaatgctcaaaactataagatagacactattattgtaaacattttagagttgacagaggtgagccttagagagatcaagtaactatccccaggtaactttggtagaaagttgaaaatctgggatttgaactaaagcctatgttttaagccactatatgacattgctcccactgtaccataggttttagtagaaatgtgggtgtaggggaacttaatgatttagatgtggctattcaagaacacttcttgttcttgtagtgcattaaatttggaatatattgaatattatcactaatctctagctagcaaccaaagaaaacaagatactcagaatagcaacagctttacataaaatactttttcaaaaatattatacattctccaataccttctgtggctctgataatttgctctcataatcagttcaatccagcttgttccttaaatgcttgagaagtacctcattttactcaacatattaccacatataaagcatgtgaaaataccagattgtgttccacttttaccccaaatagtaacaaagctcctgcaattttttaagatattattaaactgtgtacaaatgctcagattaaaaaaaagtgcttacttccattgaaattggacactaccactacctattcaaattcaagttgtcattgccttgaatccatgtgtaaagtttttggtaggatagtctatttctagttgtttttcaagactcataatttggaacattctagatataagattgcattgacactttatattctttttactttataaaatggtcatccatggtttatgttacaaacgaaagcaaaaatctgggggaaagttaaagaagtagagccagataacagaattttcttttctaatatctaataaagtgaaacaaaaggatgaaaataaaatcatgataggaaggaaaaaattaccagaaactatcaaagagagagaaaacagatctcatgccattaacttaaaatgtcacctaagaaaagaaacaatagattttgtctaggagaatgaaagccttctaaacttgtctctagaaacctgttttaaccataaactagaaaatggacatattaagttgacaaaaatcttaaaaattttctcctcatttggagaaaagtagactaaatatatattctttcattttcctcttatgaaaggagggaagttgcaatggttacatttgaaatatagatgaaaaaatggaggagaagaaaaattattcactcctcgatggaaacatagtctccagggctccatgctgaagaacaatgctgatactacattctcctcaaaacaattctgaaaatttcttgactcatgaaacccagctaactcagtagttgtaattacttacttttatgatctggtttcctttttcactctaaattcttatcctcctactcttctaaataaacaatctgttttgcttcttaaatttcaaataatttatggaaaacagaactaattctttccaactgttccttttcagatccccattcactcttctctaataacaattaaaatattattttgttttttgtaaatttattacataaatttaccatttatatatctttccttgattctagactatagttttcttgaaattaagacatatacttttcctattttaatcttcaagggccaatttagcacttgaaatatagacattcaatgcatatttgttaagtgaaaatgtattttgaagtgtaatctccttttttaaagtttcacaatctttttgactgagtccttgaaagcttgtttcacttgctgatttcttaaagtatatatgaagggattcagtaagggagtaaccgaagtaatgagtacagctattcctttgttgaaagcacctccttcttttgcagaaggattaatgtacataaacatgcagctgccataagagagggagatgacaatcatgtgggaggaacaagtggaaaaggcctttgtcctttgctgggcagaagggatcctcagaatagtcctgataatgtatgtgtaagaaagtgtcaccagcaccagagtaaccatgagagtcacaacggccaagaggatgaccatcagttctaagaggcttgtgtctgagcaggcaagctccacgagaggcccatagtcacagtaatagtgattcagaatgttggagacacagaaatctacctgggtcatcaggatgattggtggtaagattgctaggaatccccccaaccaggagcagaacactagttgtatgcagactctgctgctcataatagtcaggtaatgcaagggtttgcagatggccacataacgatcataagacatggaggccaggaggtaaaactcggtagctccaagaaatatagcaaaaaaatactgagtcaagcagccagcaaagctgataactttatttcctgttgtcatgctggtcagaaatctgggaataaaaatggatgtgaaggaaatttctaagaaggagaaattccggaggaagaaatacatgggggtctggaggtgggggtctagtaaggtgagggtgataatagtcagatttcctaggatacttagcatgtaggtgaggaacagaaagatgaatatcatcacttggagttcaggttgatttgtaaggcccagtagaataaactcaccaaacatggttctgtttttcattgttgaccttcggaaaacctgtggtctttggcaagtactgcattttcttccagattttcacagttgattcatttcatgatccacatttatagaatgataaaatcagtgactttaaaaacatatgttgctcatacctttgacaacctgaatgactatagtatactgtttaccttgttgttcctaagaggtaaatcaaagatgagatgtgccacgtgaatctttgagtagtatatactttaacatgttttctattggcttccatccacattttacctttctcttaatagaagtatccaaacttatggaacttaaccagaaaaaagagcatattattttccattctaagaatccaatccagaatcaaatcatagttcctgagagacagagaacttcacataggtaataaaaaataaaaacaaagcccatagcagttattgaattggaagaaaatactttgagagacagaaaatttctgaaaatttatgttctaagagagattatgttgaagttcttagatggcagaggatgggcatct

SEQ ID NO: 18832 - RNA, 4226 nt, Homo sapiens
  source 1..4226: mol_type = other RNA
tgcaaaagtaattgcagtttttgccattacttttagtagcaaaaaccacaattacttttctatcaatgtaatagtagaaacggggtttcactgtgttggccaggctgttcttgaactcctgacctcaagtgatccgcctgcctcagcctcccaaagagctgggattagaagtgtgagtcactgatcctggctgaaataaaaaaaattaaaaaatatattttattgttttgaattttatttaaaactctttgcaagaaatgatgctggaagactacctgtttagaattgtaatccatatatccacaagctctggcagctttaaagagaggcaatagaagaatgaatgcccaaatgtagcagattggcttttactcattttcatagtctcctcaccctagcactggtataatatgattctgagaatgttaggcagctaaagctgtttcttttaattcttgtccactttggtgacatgaggaatcaaactcaccattttatatatttagatactgaatattctggtagctcagcaccagactctgtgaagtcattccttttgcttatctatgacttggattacattccaagtatgaattaacatacagccagactagatgaacagctttagaagaatatgacttgcttttttttttttgacaagctcatttagaaggtgatacattcttttccatgttcatttccaaatgcttatataaagaatgctgagtgaactcttgcctagtgatcttaaacattaacttacacaaagtaccttccttccttgtctcagcatgttaatacatcctgtctctcccatagatatctagggcaatgaagttgatgctagcccagttcttataacctgctgccaagtattttgatggctttatctgaagagtaggtaagatctttgctgacccagctacccagcatgcagctggatgtgtggagagtagaaatatgctggccttgtgcagatggatttcaagtacaatggccaacatttttactgtccctgctatattaaaccaaccaatttaatgccttctttctagttaagctccagttccttgaaaaatatattgtttataatatagttataatagatgtcatttattaaacacaataaatactggctgtcttttaatattttacatctattttctcagtgaatgctcaaaactataagatagacactattattgtaaacattttagagttgacagaggtgagccttagagagatcaagtaactatccccaggtaactttggtagaaagttgaaaatctgggatttgaactaaagcctatgttttaagccactatatgacattgctcccactgtaccataggttttagtagaaatgtgggtgtaggggaacttaatgatttagatgtggctattcaagaacacttcttgttcttgtagtgcattaaatttggaatatattgaatattatcactaatctctagctagcaaccaaagaaaacaagatactcagaatagcaacagctttacataaaatactttttcaaaaatattatacattctccaataccttctgtggctctgataatttgctctcataatcagttcaatccagcttgttccttaaatgcttgagaagtacctcattttactcaacatattaccacatataaagcatgtgaaaataccagattgtgttccacttttaccccaaatagtaacaaagctcctgcaattttttaagatattattaaactgtgtacaaatgctcagattaaaaaaaagtgcttacttccattgaaattggacactaccactacctattcaaattcaagttgtcattgccttgaatccatgtgtaaagtttttggtaggatagtctatttctagttgtttttcaagactcataatttggaacattctagatataagattgcattgacactttatattctttttactttataaaatggtcatccatggtttatgttacaaacgaaagcaaaaatctgggggaaagttaaagaagtagagccagataacagaattttcttttctaatatctaataaagtgaaacaaaaggatgaaaataaaatcatgataggaaggaaaaaattaccagaaactatcaaagagagagaaaacagatctcatgccattaacttaaaatgtcacctaagaaaagaaacaatagattttgtctaggagaatgaaagccttctaaacttgtctctagaaacctgttttaaccataaactagaaaatggacatattaagttgacaaaaatcttaaaaattttctcctcatttggagaaaagtagactaaatatatattctttcattttcctcttatgaaaggagggaagttgcaatggttacatttgaaatatagatgaaaaaatggaggagaagaaaaattattcactcctcgatggaaacatagtctccagggctccatgctgaagaacaatgctgatactacattctcctcaaaacaattctgaaaatttcttgactcatgaaacccagctaactcagtagttgtaattacttacttttatgatctggtttcctttttcactctaaattcttatcctcctactcttctaaataaacaatctgttttgcttcttaaatttcaaataatttatggaaaacagaactaattctttccaactgttccttttcagatccccattcactcttctctaataacaattaaaatattattttgttttttgtaaatttattacataaatttaccatttatatatctttccttgattctagactatagttttcttgaaattaagacatatacttttcctattttaatcttcaagggccaatttagcacttgaaatatagacattcaatgcatatttgttaagtgaaaatgtattttgaagtgtaatctccttttttaaagtttcacaatctttttgactgagtccttgaaagcttgtttcacttgctgatttcttaaagtatatatgaagggattcagtaagggagtaaccgaagtaatgagtacagctattcctttgttgaaagcacctccttcttttgcagaaggattaatgtacataaacatgcagctgccataagagagggagatgacaatcatgtgggaggaacaagtggaaaaggcctttgtcctttgctgggcagaagggatcctcagaatagtcctgataatgtatgtgtaagaaagtgtcaccagcaccagagtaaccatgagagtcacaacggccaagaggatgaccatcagttctaagaggcttgtgtctgagcaggcaagctccacgagaggcccatagtcacagtaatagtgattcagaatgttggagacacagaaatctacctgggtcatcaggatgattggtggtaagattgctaggaatccccccaaccaggagcagaacactagttgtatgcagactctgctgctcataatagtcaggtaatgcaagggtttgcagatggccacataacgatcataagacatggaggccaggaggtaaaactcggtagctccaagaaatatagcaaaaaaatactgagtcaagcagccagcaaagctgataactttatttcctgttgtcatgctggtcagaaatctgggaataaaaatggatgtgaaggaaatttctaagaaggagaaattccggaggaagaaatacatgggggtctggaggtgggggtctagtaaggtgagggtgataatagtcagatttcctaggatacttagcatgtaggtgaggaacagaaagatgaatatcatcacttggagttcaggttgatttgtaaggcccagtagaataaactcaccaaacatggttctgtttttcattgttgaccttcggaaaaccttgttgttcctaagaggtaaatcaaagatgagatgtgccacgtgaatctttgagtagtatatactttaacatgttttctattggcttccatccacattttacctttctcttaatagaagtatccaaacttatggaacttaaccagaaaaaagagcatattattttccattctaagaatccaatccagaatcaaatcatagttcctgagagacagagaacttcacataggtaataaaaaataaaaacaaagcccatagcagttattgaattggaagaaaatactttgagagacagaaaatttctgaaaatttatgttctaagagagattatgttgaagttcttagatggcagaggatgggcatct

SEQ ID NO: 18833 - RNA, 65 nt, Homo sapiens
  source 1..65: mol_type = other RNA
tgcaaaagtaattgcagtttttgccattataatggcaaaaaccgcaacttaatggcaaaaactgc

SEQ ID NO: 18834 - RNA, 4559 nt, Homo sapiens
  source 1..4559: mol_type = other RNA
tgcaaaagtaattgcagtttttgccattatttttatttttattttttatttttatttttttcaagacagagtcaagtgctgggattacaggcatgagccactgcgcctggcctttgccattacttttaatggcaaaaaatgcagttaacttttacaccaacctaatagaacgtaaagcagcttaaaacaagctgccctgactcagcagttcccaacaacaatcattcatctagaactacccaaggaaagcaacaaaaactttaattcccttaaggtttagaaccaatacaatgctcaaaggtctctgtgcaggaaaaaaaaatgcacagcaaaaagaaaaccttgctaggtacggtcgcttatgtctataatcccagcactttgggaggcccaggcgggagaactgcttgaggtgaggagttaggagatcagtatgggtaacacagtgtgactccatctccacgcgcaaatttttttttaattagttggacatggcgacgcatggctgtagtcccagatactcaggaggctgaggccagaggatcacttgagcccaggaggtcgaggctgcagtgagctatgattgtgccactgtacttcagcctgcgagacagagtaagaccttctctcttaaaacaaagtcacaggttctgagggttagggaaaaaataataaatttaataaagaaaaaagaaaactcaaaaaacaaacagcatttgcttcctatgaaatatttacccctttaccctaaatttaactgctttccagtccaaagctctacacacttcatgtgggcctttataaagcaaccactggctttatgatttgtctagaatacttgaagaaggaagtttatgactttgtcaaaaagctgttgtatattcccacttaacggataaataaagcaggttctattcaattggaagaaacaggaataaagacgtgtgcattttcagatttcctttgagtgccctggccttcagaccattcagtgtggcatttaactagtttagattatggttattgttgatcctctatttactgatgttccatgccttttatgaagaaaaatagctacctaattctctttcacccagtgaactatatattagagttgttgttgtttaattggaacagaaaaatagtttgatgaacaagctctatttttcttacccccaaattaattaccatcacttcaaggaagagagagggcaccaactctatttggaagctattttacgatctagactcccccacacacagtatcataggtgtctcatgtggatcacagaacacaggcaacataacaccagttgtagaggaaaagcctggcagagattccaagaacagcttgtctggggagtcctatggcagtaggccaagcaggaagaccatcgcggtaccttctggatggaggtactttcaaaccgggaggcccatccacatttcagattccactggagttctaagacctggtgtaacaggttctggtagccaacgacaatcccagcctaaaagtaggatttggcaatacagataacattcactctcttctggggcctagcaactcttcaacttttatctgtagtaaaaacagatgccaaatattttagctaacctggaatcaatgaaatatcttctcttacacttgtaccactactaataaggaaaacagataaaggggcatatgcattagatggtaccacagaaccctgaattcaactcggacccaagcaaaaattgaagccatcatcctgattataaaacccagtgagcttgatgcagaaagccactcctctctaggaataatcatgtcctatcacatagggactagcagcaagactgatttatccatgctaacggagggtataaatactcaaacccagaaaaaaactctggtatctgactccaggtctaaaggccagttgcccagggcatacaccacttacacagaaatgggtttccaaaggctacattgaacagccccacatctgctaggggatatgaaactgttcaggtccataggggctgaggtgttgcttgttttgcctcagctttccctaagctttcactgaccagctatcataggtatgagcgtggggacctaagttcaacctggctagagagcaggcaagccttcttaaagcgcagaggctccacagtcattagctaaggcagcaacgcctcctgctcaccagtgttggggaagagacttttgccttaggccagctgattgattacagtagttgggccaagtcctgaactgcatttccacaatgcaataataactactgcaagcaagccattatctggctaatttcctaaaattaaaaaaaaattttgttgttgggtgtggtaagggaggggtggtcctcactatgttgcccaggctggtcttgaactcctggcctcaagtcatcttcccactttggctaagtgctgtaattacaggcatgagccactgtgctcagccctaaaatattgttagagaacatttacagacataaagatgagctcagtctcatccttatcaatctcctaaaaggaaaatttaagatctagtacttataatcctgtcctcaaagcaaacctaaaaataactgtctctctgatttgttttacagaatcatttatagttgtgtctgtcaaatagcaagaatcattcctagccagtgatgtggttatcacttatcttatgtgagggtaaacctgcaatatcttagagtcctttctaaaattatacagaagtcaaaataacctttccaaaaaggagtactaaaaaactgtcactgatagaaaacatcaactgtatgccaaagtactaaaaaacaggcaatcattccatttcagttgtattcacctattttcatcagtaggcagggcagtgctatcagaagagtaggctgcccttctatgacgacagaagctgttcctgatacttagttctgccttgcacatagtagactcaggtatcagtaaaatgaatgaatgaattatgaaatacactgactggtgagtcagacgttttttaacattccaggaaaaaaaagaaggctgaaattcctaatgaaaaaaggatgtctcattgagagatttttgcattactctttctgtatacgaaagcttgttgtttagataaattaccacaacacaggactttcacatacctgtctttattttgcttttatttgtgatttgatttaaataaataagaaggttcacacaggttaataaaaagacaagcaagtttgttgtatggctgagaaataatatgctctcttggtgtatactgatggcattatcggataacaccatgaggaccctcctcttcctcatttcctgggtcagtcctggtcagtgcttcttccgcctagtgctccttttgtatcacttatgtacactggatggagagaaaagaactcttctatgccttagtcaacatagatagcagcaggtgagaaaaagagctgatttctgatgtaacagaagcagactgactcctgctagctccagatacaaaatgctctacaggatgacttactgtaagtcactactgataagttgtttgcgtgactgctgggagacagatttacagagttctgtgacagtctattctggtcttgctcagtttggtcaggagcaggagcccatgtgtcaggagcaggagcccatgtgtttttgctgatcgagtcgaactcggagcccccagggtcttttaagttgttttcatctgattgtcggttcttttggggagaggcaaaagggttgaagtttccttctaccttacgatgcggctgtgtgttgaactccgtttcaaaagatgacagctgctgcgttactcctaaaagtccacccacctccacactgagaatcacccagatgacatctccatagtagagtcctgtagcagtgcacatccgccactgtccctgatacattcctgctctgctggggctgcacatctggacgctgacatctgcaatctcttggggctctagcgatctcaccatcaccatgttcacatgtccaaattggtctcccccgacatatttaagacaaacccctggaggccaggcctctgccccagaattctggatccgccatgtttttacaaactgagtatccggaggtattgactccccttctcctatggtgacatcttcaacaaaggacatagagggcacactgatgtttgggctctcaaagtcataataggcgccaattgctgcttgtaggttccagttggtcatgtccaggaagaaggcgcaaccggcaggattgagctggaagccgagcagcctctggaactcggagatgagcacgtccttgtcggtggtgcccaggcagctgaacttctgcatcagctccgggtccaggtctacgtccatgccctccatggcggggaccggacacccgcttccccgcctcttcacaaccaagccgccgccgcgccgccgggcccggggacctggaggggggccgctgctagctagcttcgcgaccccgctcctttgaggtaggccccgggcctctcacagtctcataggggtaaactcact

SEQ ID NO: 18835 - RNA, 4897 nt, Homo sapiens
  source 1..4897: mol_type = other RNA
tgcaaaagtaattgcagtttttgccattgaaaataatggcaggggagactcttgatcttatcattcaaggctttctgttgctcaatgttatattaaaaacaatgaatttccatactaatttcaaagtcaattcctaagatactgtttcatcccattgtgaacaccaccaaggtcagttatatgtttttcagaatacttgaagtacgagaaaaacagaaatatatagctctggctacattaaatatcttttgccactttctgagatctttcgtaactctaagagaaacatggcatttccattaacgaaaataggagctttttgaataggattgttcaaaattagatacaaatgttctcagctaaaggtctcacatattcagaagtttgggtgccttttgtgatagctcttgtatcatttgataatattgatttttttgaaaaaggcaggctatttacaaggcaaagagtttttgttttgttttgttttgtttttgagatggagtcttgctctgtcgcccaggctggagtgcagtggcgcgatctcggctcactgcaagctctgcctcctgggttcacgccattctccggcctcagcctcctgagtagctgggactacaggcacccgccaccacacctggctaatttttttttgtatttttagtagagacggggtttcaccatgttagccaggatggtctcgatctcctgaccttgtgatccgcccgcctcggcctccaaaagtgctgggattataggcatgagccaccatacccagcaggagtttttaactttcactttctcaagtagagaaggccctcaactgtaaacccctttaccctagtctctgggaaatattcctgcccaccaagcactctatcccccccagcccccagctccactgggttattctagggtgagggagcggacatgatcatccagtagcgtctgaccagccggaaggcaaaagagacaagcaaaagttctgtgttacccaggagagctcagctgtccagaaataattagagctacagccacacgtggttcaaggaaatgtggttgtcagagagagacagagatctgccaagccatctcctcttcaactgcctgggcggagggggctgcagcccacattttagagacacagtattgtttgcagttgatttagaacttgagctggaagaagtcccccatcatgacctgcacaccattagaagaaagtgttgtctccaacaagctcagccacaatgttggctgccaacggtatgtctttccccactcattggaaaggagattatcacactaaagcattgagatgaattccgatgaacaaaggtagtcagaccgttaggctggactgtcactaggacatgatgacaatgaataaacttaggctcttgcaatgtccatcactgacatgttttaataagagttgaacgcacaaattggcttccttgcaatgtttacttcaagcagtaggtctgtctgctctggcctttgatgggatctgccagcttcctccctccttgtctatgtcccctgccttcaccatgggaaaaaaggctccagtaaaccaaatcccagaagtgatgttgcctgcggagaccaactcaaaaccaactggcctcccactgcttcctttgaaaacatatacatttcacacacctgagtcctcccacccctctccactccacggcaggctccatgaatggaactccaggggctgcctttgtgtaatgatcaagacgtccctggacagaggagcagcttcgcatcagggaatcctggtcccctgatccccatgggatgagatggtgggtgtagcatccttctggtttctctgcccattcagctgtctacccatgcacaaaacccaaagccctggattttggattttgtacctgcaaacctgagtaaactttttcccctcaagagtcatcattcaggccgggtgcagtggctcccacctgtaatctcagcactgtgggaggccgaggcgggtggatcacttgaggtcaggagttcgagaccagcctggccaacatggtgaaaccctgtctctactaaaaagtacaggtgggcacctgtaatcccagctactcgggaggctgagacaggagaattgcttgaacccgggaggcagagttgcagtgagccgagatcacgctactgcactccagcctgggcgacagatcaagactccgtctcaaaaaacaataaaagtcaccattcagcctgaccaaggagggggccaggaaagaagtcggaaccgtggccttcgctgcttcagaaggggaggcccgtgctctgacttcagcttgattcactttggcctcagtcctcagttcccagggggtaacggcgttctgaggttgtcacctggtgcaagaccagctgtccccagggacacatctggatctcttggtgccaacaacggcaactccagagggggctgggtgggggcatgtggctccagtttgaatgcaccatgtccatctgccagagaatccactggtcaggctctagggaggcaaaccggggggcccctgccaggaaatagctgctcagaccacacctagatcgcctgcaatttcaaagaagaaagcctggggctgtgagtgtgggagaaacctactgaacaggtccggtgggtggacagcaggtgtcacatgggcctgagcctggacggtatctacagagagatattttggttgttcactgagggtttggccgggtgactctgggtggtgtctgattggttgctggcattaccagaccctcctaatatgggtagtcttcccatgtagatccacaggttatgaacaaagctttcaccacatatacagagaaccccctagagcaaacatctccccatccctgggtggacctcaatgaagatgagcaaactgagtcaagacacaaaaccctgttggtccaggtcatactcttgggtgagttcttgatgtcggcagtgacaatcagtgccccagttggggcctgccagccccccaagctctgcagcctcaaagaccagctcagtcccccatcggtcactattcctgagagccagagttcgacctggtaacacctgcaccgtgcattcctcggccgaccatctcctggccccactcccggtggctggactcctgcagtcctcggcctttggtctcaatgggcaaaaagcaggaggccagggcagccaggaggcagcagccactgtaaactgccagagtcaggtacacagaggattccagcatcacctgggcgatgaacggagtgatgagagcacccactcttgccatgccgctgcaggtgcccaggccgagggcccgcgttgccgtggggtagacctcaggtgtgtaaacatatgccgcttgaaagcctccagaaataaacgctcttgcaatgaagagtaacagagtgagcacatttcttccaacacagataaacagcaggaggctgcagaaggagaagatgacaaagcacagggccatggtcttcttgcgccccaggcggtcaataatccacagagtcacaaggacacctggaaactcagagagggtggtccacagcaagtccatgtaatcctcctcactcaggtactcgcaggccaggctgcattttgcctctacagccttcttccgactggagatgccgcagacatctcctgcctggaagagttctgtggtgagtagaactaacccgtagtaagagaatgcattggaaaaccatataaaccacagcagcaaagttgtccatctaaaatggggtgtgaaaaggtccctcattttgcctcggtcttcctgtctggagatgatgagtttccccagcggcatgggagctccgttttcagttgctatcctctttaaggtggcgattgccttttcctggttccctgacagcacatcataccttgcactttcaggcagccagaaacacagcacggcaaagaggaggagcgggacagctgagaggatgagcagccaacgccagcccaggctgggcatcacgaacacagccaggacgacctcgaacactgtcccgatggcccagaatacctcaatcagcaaaatacatttagctctggctttcatgggaaggaactcggcatacagcgtcaccgactggggaactcctccgatcccgaagcccaccaggccccggagcaccaggatccagctatacacgggcgcaaatgcactaaggatgccatagtacagagtccacagcacgctgatcttcagccctgttttcctgccgtactggtctgagatatttccccagagcgtggagctggacatcatgcctacaaagaccaccgaggtcagcaatgccacctgccagcttgggagcctccactcgcaatgcagctgtggtgccaggatgctgaggatcatcatctccatggcatcagccatccaagccaagccagtgagaacagacagcttccactgaaattttccaaagccaatggcttccactgcatcttccaccatgaaagtatcatcagtgggattggcaaactccttgggcacagctgccccatcatccagctccacagcctctaggcccacgtggaccccttcaatctggacttcatgctctcctgaagccgtgtcgtcctctgaccttgcactctcgcctgtgcgacggaatttcacaaccggcagctgccttagctggaataagtcctcctccatgtccgcgctgcgccaggatgagcccttctcatggcccttacatggtagtggtggatgacgagccctccggttttcagcaccgggaagctggacagcacccgcgccgcttcctccctggagcagcagctgttcggggagggagccgctggggaccagcccacgagacaaagcctccgccgccaggagaccgcggcgagagt

SEQ ID NO: 18836 - RNA, 415 nt, Homo sapiens
  source 1..415: mol_type = other RNA
tgcaaaagtaattgcagtttttgccattgaaagtaatgtcagttacttttgcaccaacctaatacaaaccatcccatatctgtgttctccatcctttcatcctttatcacagtggggttgtgatagatccctgaaaacacaggatcaagtataggtaaatgcaagatggtacatagaatcaagtgtgaaagtgagtcccatcaacccacactctttccatttggcccagttgctgcccttgttgtttagaatggcacgtacctggccttgaaatgcactgaagcctatggggattactttaaaattcggtcctgtaagccagtctgttagtatcattgctcctactaatgatagaaattgctggtgttggccgggtgtggtggctcacaccagtaatccaagcactttggcagac

SEQ ID NO: 18837 - RNA, 87 nt, Homo sapiens
  source 1..87: mol_type = other RNA
tgcaaaagtaattgcagtttttgctattactttcaatgacaaaaaccgcgattacttttgcaccaacctaatacatgcagaatcaga

SEQ ID NO: 18838 - RNA, 7559 nt, Homo sapiens
  source 1..7559: mol_type = other RNA
tgcaaaagtaattgcagtttttgtgattacttttaataaaaacaaaaaacaagaagccacatggcagcaaaagaagtatgccttctgtatctgaggatgttgctgatagagctagcaagatagaaaaatttgtattataataaatgatttgtaataattctaagcacccaggaggtttacaacagtgattctaggtagcacattaagaactacacacatattctttgcaaagaagaaaaaatgtttatgattaaacttcgttagttttcttccctgaatttaatacttttccagaattaaaacagaagaactagcactatcctgagccctagatttaaccttccgatgtccagaaattcattacaatagaaagcaaagtgattgttttcctttctgtaattagctttccctgctatatttttcgacaggcaatattctaattgtgctaggcttgccattccatttctggcatagttagagtgattttaagtttactgctttagtgataagttttttagttcgggctcaataattagcacctgaacatggaaaacattaaattaaaaaaatggaaatttaccaaagtatttgtttataaaaattatagaattcacagaaacgtctttagcttctctagtcttcagtagttatatcatttttatagaaataacaaagtattagtatattactcaacagtaatgaaatatttctgaatgaaaactgtgtagcccttatttaagtacctaatttgaggttttcctttccattgtgaaatagtgattttgctttgaaaaataattgagattagtttgctgatgcaatatttttctaccactgtctcatttcgattttaaataataaagctaatggtgtgtctctcaccaatactgagctctacaaacctatgtgtctcttactgaagagcttcgttttgaaattactttatctattattataattggtacagtttaaggttttgtctttagagaattttttaaaggttttaaaatctattttaaatggggctttttagtataaactggacacaaggaacacttcagttcatgggataactttttttctctattaaggtgttcccttaattctaaagtaaaggcatggtagcaagtttaaaagagaggtcaagctgatctacgatgtgattttttaggcttctggttaaaaatagatttatggctatgttaataaaatgtgcatttattatttctacatatttttttaaaactaggcatttcataggtgtaccataatgactagttaaaaatggaatcaaagtgaagtgaacaaatggcctaagtattctttgaaatatggcagaatataagtaccttaggtgacgaaaggacagccaagacagcgtgaaaggaaaacatataaaatgtacaaggcactggagagaagttatacatgatcgctgccttcataatagattcattgatatacaatgtgaataagggttgacaaataccagttgaataaacaattattaaaaagtttcaagtggaagcctcccatatttctccactatatttttgcaagtgcttaacaaaacaaaacaaaacaaaacaagggtttagggtggggaggggaataaaacaataatcaaaagtctcccctaattatcacagtcaggcctgaattagtaaccttgaatatcaaacacaaactctcaaagtataggacagaaacaacaaaacaagtaattattaagcacctactacatgccaactacagttctaagaattgaaacaaaacaaaacaaaaagggcaaggagaaacgaaaagataagacaatgaaagagaagtcgaagtcaggcccggcacggtggctcacgcctgtaaatcccagcactttgggaggccgaggctggtggatcactagagcccaggagttcaagaccagcctggccaacatggtgaaaccccacctctgctaaaaaaaaaaaaaaaaaaaaaaaaaaaaaattagccaggcgtggtggtgggcacctgtaatcccagctgcttgggaggctgaggcaggaaaattgcttgaacctgggaagcggaggttgcagtgagctgagatggcgccactgccctctagtctgggtgacagaatgagattttgtctcaaaaaaaaaaaagggaagaaaggaagaaacatagagaggtcagttacatgcaatttttagataatccaaaaaagaagaaggaaaaaggagaagcaacaattagacaaatattagaagaaaatatacctgagctgagaaaaggtttggaccttcattgaaagagctcccaagaagtctaagaagtgacggaagagaataaaaaaagacatcagatttcttgacgagattaagaaactgtaagtttttacttttttcttttaaacctcagtttacaagcttccagctgtaacgaatgaattccctacaaagggaaaaaaaaccaaagtggctttggaattctcaactgcaataccagaagctagaaaaaagtgggcacaatatctatagaccaacaaaacaaaaggactacaacccaaaaatcgtatacccagctaaactatcatttcagaggggaaaaaaaagatgatattcaacaactaaattgtacaaattgtacaccaaaatataccaagaaaaatatagtacagttccaagtcttcactaataaacatgtagccttgaacaggggaccagctgaaaacaactgggggacattcacaaaatgcagtatgatgcagttaacaaaaagaataactttgttataacaaatgacagagagggatttatataagctgtaactgcaaaatataatttaaaaactttgtatatcccagttctgcaaaataaaaatacatcccctatatgtctgcatagatatatataggattgcaatatgaaagaacacagtctaggttaataacttggtttgtggcagcaggggtaaggactggggaatgtggtactaatgtggaaagagaggggtgtttataacaacagcttgttgaacatcccattatgtaaaattatatgtatcataagagattcatgaagaatgaccatgaaaatgttagtggtggttaccttatggtattataattccaggtgaccactaccttcctttttagatttttatgttgtttgaattatttataatgagcctatatatctatataactagaagtaagtaaaacagttacttgcagtttggaagcagacttcctttttcttaaaaataaatttccaattttaatagcttttcttttctttttcttttgggagacacaaggtctcgccatgtcacccaggctggagtgtagtgacacgatcttggctcaatgcagccgtgactttacaggttcaagtgattccccagcctgagtctcccaagtagctgggactacaggtgtgcacaacacacttggttaatttttgtattttttatttagagacgaggttttgccatgttgcccaggctggtcttgaactcctgagctcaagtgatctgcctgtctcagctcacaaagtgttaggattacaaccaccgtgcccggccaatagctttttcaaactagctttttcaaaggtcaaatgcatcctcaccaaggggacaagattgaaagtagaatggcctgggcttaataaatcaatgatttgaaactatcagaagaaaacatggagaaaatgctccatgacattggtctgggcaatgatttttttggatacgatctcaaaagcacagtaacaaaagcacaagtacagaaatgaaattacatgaaactaaaaagcttctgcacagcaaaggaaacaattaatagggtgaagagacaacctacagaatggagaaaaaatattaactatagatctgatagggggttaatatccaaaatacataaggaactcaatagcaggaaaacaacccatttaaaaatgggcaaagaacctgaaaagacagttctcaaaagaagacatgcaaatggccagcagatatatgaaaaaattatcaacatcagcagtcaccagggaaatgcaaattaaaacaacgagataccacctaacacctgttagaatggctactatcaataacacaaaagataacaagtgttggcaaggatgtgaagaaaaaggatttcttgcattattgtgaagaaaaaggaattcttgcatattcttggtaggaatgtaaattagtacagccattatggaagacagtatggagtttctgcaaaaagttaaaaatagaactacatatgatccagcaatcctaatactgggcttatatccaaaggatatgaaatcagtatgtcaaagagatatctgcactaccaggttcactgcagcattattcacaatagccaggatatggtatcaacctaagcatctgtcaatggttgaatggataaagaaaatgtagtacatatacacaaacagctgatctcatagaagtagagagtagaatggtggttaccaggagctagggttgttggagaaacattggtcaaaggatacaaaatttcagttaaaaagggggaattagtgcaagagacctattgcacaacatagtaactatagttacaattacaagattactattaattttgaaaaataagagaatggatgtaaagtgttcttaccacaaaatggtaaccatgtgaggcatatgtcagttagctagatttagtcattctataatgtatatatgcttcaaaacagtatgttgtacatggtaaatacatacaattttatctgccaattggaaaaaaaaatcaattgtaaaagcaagtgtttggaaaacatttagctggaaaggtctgataggaggtctaacccttatacacttaaaaactcaacaactggctgggtgcagtggctcaagcttataattccagcactttgagaggccgaggcgggtggatcatttgaggtcagcagttcgcaaccagcctggccaacatggtgaaaccccatctctactgaaaatacaaaaaaattaaccgggcgcagtggcgggagcctgtaatcccagctactcaggaggcttaggcaggagaattgcttgaacctgggaggtgaaggttgcagtgagctgagatcaaaacactgcactccggcctgagcgacagagtgaaactccatctcaggaaaaaaacaaaaaaacaaaaaaccctcaacaactgtttacttttggtattcaagctcataaaagcctcatttactagtctactgctggtaaggatcaggaagggaaaattaagattaccttcatgataatcacgtgtgggttgacacagacggagacaataacatagaaattttattacagcatttcatgtttaagccagattccctgccaggatattttctgcttgaattaatgaggcaggatttggtcataccttaatgagtttcacagaaaaagagttcaagcattagcgcaaactgccttctgacattaaaataaaataaagcaaacatgggattttcacaaagttaaaagcctcctgtgatgcacattttggatagtaggagacattgagccccaaaatgtttaacataaagcatggttaattaaatgaaaccactgaaaaatgtgaatacatgaagaagaaagaataaaataattttgatgttaccatttcaactactatttttgatataatcattcttggcaaaatcattcttaaaggtggaaacgagcaggctgatagtacagcaagtaagagaaagtcaatactgatggcctccacttgctgatcctctgagactgcatcttatagttcataaaatctgctgaaggtcacaactgaggtacaacgacttgtgttacttgtactgtagcaatgagggctttcccaggccacaacatctgggatcaaggaacacattttgactaaataaactatacagaagtctgttttaggattttatgcaaatattaacctcattttaaaacatgaggaaaaatattacccacatttagggctaatttagctgtcaggaatagaccatacagttgaaaaaaacacagtctcatttaaaaagtttcagcagagacaaaaaggtactaaagatgatattcatccttcttcatcactgctgctccaggcatcttcaaaggccggatttaattgtgattttgttgtagtctcatcatcatcaggaactggttcatataaggatggaacccaagccagaatgttgcagtctctgctaccactataaagttcctggaaatttgactgaaatacacagcagtcaacagttttataatgtcccttaagcatagttatctgttctcctgagtaaactgtataaacagcaatggtgctaccatatggtacaaaaacaaattctgaactgcagccacaggagacagtgaatttcaatccttttttactgttattacaaacttttccatagttcacaagtgtgttttctccattggaactattccagagcctcattcgattatctgtaccaacagtgaggaggtgaagtccatcacttgtaaaacataagccattaactttcccattatgagcagtgtttgctgattcaacagcttgtgactttttcccattatgttgatcaagagtaatcaaacatcctgatgctcttctcacatcccataattttactctactgtcagcacttgctgttgccaagatatagtcataacgtggagaccaggaaactgctaatatttcttgtctgtgaccctgtagaatgtgagaacaggatccagacttcaagtcacaaagttgtactttgggtcctctagtaccaactgctaccaaacagtgcttggtggagactggagacatatgatgactataaactgtttcctcaaaattaaatacatctgcagtttgtaatgtatttgtatcccatactttcagagttttatcaaatgagcttgatgtgaacatgccagtgtcatgaggataccactgtacagtctccacactgtatctgtgaacatcaggatgatctctgccaatggaacacactgctttacatgtgtaataagattgtctgctggagttctcaaggtcataaagtacaatcacaccatctgaaccacctgataacatgcgtcaatccttaagttgctgtctctcttgtcattctggttgaatgatttcattctctggttgattcctaaggaatggctaatgagaacaacagtctctgaattcttgtgttgttgacaatttatccgtcctttttgtatctgaaatcagtttggctggatataaaatccttgactcacattttatttccttgagcatcttggataagaagcttcattttatctcccttcaacaggttcaatgtcaagggtgttaattccaccgccgtggattctttcaacatctctgtctttatttaattccagtcccaaaactctccgtgttgactctgctctccgaaggcgaagagggtcctccaaacccgtttggcgtgcggacaaaaaccccagcatatcgtgtcctcacaccggctggagcactggacgtcgccatgacagagctcaggggcgggact

SEQ ID NO: 18839 - RNA, 7341 nt, Homo sapiens
  source 1..7341: mol_type = other RNA
tgcaaaagtaattgcagtttttgtgattacttttaataaaaacaaaaaacaagaagccacatggcagcaaaagaagtatgccttctgtatctgaggatgttgctgatagagctagcaagatagaaaaatttgtattataataaatgatttgtaataattctaagcacccaggaggtttacaacagtgattctaggtagcacattaagaactacacacatattctttgcaaagaagaaaaaatgtttatgattaaacttcgttagttttcttccctgaatttaatacttttccagaattaaaacagaagaactagcactatcctgagccctagatttaaccttccgatgtccagaaattcattacaatagaaagcaaagtgattgttttcctttctgtaattagctttccctgctatatttttcgacaggcaatattctaattgtgctaggcttgccattccatttctggcatagttagagtgattttaagtttactgctttagtgataagttttttagttcgggctcaataattagcacctgaacatggaaaacattaaattaaaaaaatggaaatttaccaaagtatttgtttataaaaattatagaattcacagaaacgtctttagcttctctagtcttcagtagttatatcatttttatagaaataacaaagtattagtatattactcaacagtaatgaaatatttctgaatgaaaactgtgtagcccttatttaagtacctaatttgaggttttcctttccattgtgaaatagtgattttgctttgaaaaataattgagattagtttgctgatgcaatatttttctaccactgtctcatttcgattttaaataataaagctaatggtgtgtctctcaccaatactgagctctacaaacctatgtgtctcttactgaagagcttcgttttgaaattactttatctattattataattggtacagtttaaggttttgtctttagagaattttttaaaggttttaaaatctattttaaatggggctttttagtataaactggacacaaggaacacttcagttcatgggataactttttttctctattaaggtgttcccttaattctaaagtaaaggcatggtagcaagtttaaaagagaggtcaagctgatctacgatgtgattttttaggcttctggttaaaaatagatttatggctatgttaataaaatgtgcatttattatttctacatatttttttaaaactaggcatttcataggtgtaccataatgactagttaaaaatggaatcaaagtgaagtgaacaaatggcctaagtattctttgaaatatggcagaatataagtaccttaggtgacgaaaggacagccaagacagcgtgaaaggaaaacatataaaatgtacaaggcactggagagaagttatacatgatcgctgccttcataatagattcattgatatacaatgtgaataagggttgacaaataccagttgaataaacaattattaaaaagtttcaagtggaagcctcccatatttctccactatatttttgcaagtgcttaacaaaacaaaacaaaacaaaacaagggtttagggtggggaggggaataaaacaataatcaaaagtctcccctaattatcacagtcaggcctgaattagtaaccttgaatatcaaacacaaactctcaaagtataggacagaaacaacaaaacaagtaattattaagcacctactacatgccaactacagttctaagaattgaaacaaaacaaaacaaaaagggcaaggagaaacgaaaagataagacaatgaaagagaagtcgaagtcaggcccggcacggtggctcacgcctgtaaatcccagcactttgggaggccgaggctggtggatcactagagcccaggagttcaagaccagcctggccaacatggtgaaaccccacctctgctaaaaaaaaaaaaaaaaaaaaaaaaaaaaaattagccaggcgtggtggtgggcacctgtaatcccagctgcttgggaggctgaggcaggaaaattgcttgaacctgggaagcggaggttgcagtgagctgagatggcgccactgccctctagtctgggtgacagaatgagattttgtctcaaaaaaaaaaaagggaagaaaggaagaaacatagagaggtcagttacatgcaatttttagataatccaaaaaagaagaaggaaaaaggagaagcaacaattagacaaatattagaagaaaatatacctgagctgagaaaaggtttggaccttcattgaaagagctcccaagaagtctaagaagtgacggaagagaataaaaaaagacatcagatttcttgacgagattaagaaactgtaagtttttacttttttcttttaaacctcagtttacaagcttccagctgtaacgaatgaattccctacaaagggaaaaaaaaccaaagtggctttggaattctcaactgcaataccagaagctagaaaaaagtgggcacaatatctatagaccaacaaaacaaaaggactacaacccaaaaatcgtatacccagctaaactatcatttcagaggggaaaaaaaagatgatattcaacaactaaattgtacaaattgtacaccaaaatataccaagaaaaatatagtacagttccaagtcttcactaataaacatgtagccttgaacaggggaccagctgaaaacaactgggggacattcacaaaatgcagtatgatgcagttaacaaaaagaataactttgttataacaaatgacagagagggatttatataagctgtaactgcaaaatataatttaaaaactttgtatatcccagttctgcaaaataaaaatacatcccctatatgtctgcatagatatatataggattgcaatatgaaagaacacagtctaggttaataacttggtttgtggcagcaggggtaaggactggggaatgtggtactaatgtggaaagagaggggtgtttataacaacagcttgttgaacatcccattatgtaaaattatatgtatcataagagattcatgaagaatgaccatgaaaatgttagtggtggttaccttatggtattataattccaggtgaccactaccttcctttttagatttttatgttgtttgaattatttataatgagcctatatatctatataactagaagtaagtaaaacagttacttgcagtttggaagcagacttcctttttcttaaaaataaatttccaattttaatagcttttcttttctttttcttttgggagacacaaggtctcgccatgtcacccaggctggagtgtagtgacacgatcttggctcaatgcagccgtgactttacaggttcaagtgattccccagcctgagtctcccaagtagctgggactacaggtgtgcacaacacacttggttaatttttgtattttttatttagagacgaggttttgccatgttgcccaggctggtcttgaactcctgagctcaagtgatctgcctgtctcagctcacaaagtgttaggattacaaccaccgtgcccggccaatagctttttcaaactagctttttcaaaggtcaaatgcatcctcaccaaggggacaagattgaaagtagaatggcctgggcttaataaatcaatgatttgaaactatcagaagaaaacatggagaaaatgctccatgacattggtctgggcaatgatttttttggatacgatctcaaaagcacagtaacaaaagcacaagtacagaaatgaaattacatgaaactaaaaagcttctgcacagcaaaggaaacaattaatagggtgaagagacaacctacagaatggagaaaaaatattaactatagatctgatagggggttaatatccaaaatacataaggaactcaatagcaggaaaacaacccatttaaaaatgggcaaagaacctgaaaagacagttctcaaaagaagacatgcaaatggccagcagatatatgaaaaaattatcaacatcagcagtcaccagggaaatgcaaattaaaacaacgagataccacctaacacctgttagaatggctactatcaataacacaaaagataacaagtgttggcaaggatgtgaagaaaaaggatttcttgcattattgtgaagaaaaaggaattcttgcatattcttggtaggaatgtaaattagtacagccattatggaagacagtatggagtttctgcaaaaagttaaaaatagaactacatatgatccagcaatcctaatactgggcttatatccaaaggatatgaaatcagtatgtcaaagagatatctgcactaccaggttcactgcagcattattcacaatagccaggatatggtatcaacctaagcatctgtcaatggttgaatggataaagaaaatgtagtacatatacacaaacagctgatctcatagaagtagagagtagaatggtggttaccaggagctagggttgttggagaaacattggtcaaaggatacaaaatttcagttaaaaagggggaattagtgcaagagacctattgcacaacatagtaactatagttacaattacaagattactattaattttgaaaaataagagaatggatgtaaagtgttcttaccacaaaatggtaaccatgtgaggcatatgtcagttagctagatttagtcattctataatgtatatatgcttcaaaacagtatgttgtacatggtaaatacatacaattttatctgccaattggaaaaaaaaatcaattgtaaaagcaagtgtttggaaaacatttagctggaaaggtctgataggaggtctaacccttatacacttaaaaactcaacaactggctgggtgcagtggctcaagcttataattccagcactttgagaggccgaggcgggtggatcatttgaggtcagcagttcgcaaccagcctggccaacatggtgaaaccccatctctactgaaaatacaaaaaaattaaccgggcgcagtggcgggagcctgtaatcccagctactcaggaggcttaggcaggagaattgcttgaacctgggaggtgaaggttgcagtgagctgagatcaaaacactgcactccggcctgagcgacagagtgaaactccatctcaggaaaaaaacaaaaaaacaaaaaaccctcaacaactgtttacttttggtattcaagctcataaaagcctcatttactagtctactgctggtaaggatcaggaagggaaaattaagattaccttcatgataatcacgtgtgggttgacacagacggagacaataacatagaaattttattacagcatttcatgtttaagccagattccctgccaggatattttctgcttgaattaatgaggcaggatttggtcataccttaatgagtttcacagaaaaagagttcaagcattagcgcaaactgccttctgacattaaaataaaataaagcaaacatgggattttcacaaagttaaaagcctcctgtgatgcacattttggatagtaggagacattgagccccaaaatgtttaacataaagcatggttaattaaatgaaaccactgaaaaatgtgaatacatgaagaagaaagaataaaataattttgatgttaccatttcaactactatttttgatataatcattcttggcaaaatcattcttaaaggtggaaacgagcaggctgatagtacagcaagtaagagaaagtcaatactgatggcctccacttgctgatcctctgagactgcatcttatagttcataaaatctgctgaaggtcacaactgaggtacaacgacttgtgttacttgtactgtagcaatgagggctttcccaggccacaacatctgggatcaaggaacacattttgactaaataaactatacagaagtctgttttaggattttatgcaaatattaacctcattttaaaacatgaggaaaaatattacccacatttagggctaatttagctgtcaggaatagaccatacagttgaaaaaaacacagtctcatttaaaaagtttcagcagagacaaaaaggtactaaagatgatattcatccttcttcatcactgctgctccaggcatcttcaaaggccggatttaattgtgattttgttgtagtctcatcatcatcaggaactggttcatataaggatggaacccaagccagaatgttgcagtctctgctaccactataaagttcctggaaatttgactgaaatacacagcagtcaacagttttataatgtcccttaagcatagttatctgttctcctgagtaaactgtataaacagcaatggtgctaccatatggtacaaaaacaaattctgaactgcagccacaggagacagtgaatttcaatccttttttactgttattacaaacttttccatagttcacaagtgtgttttctccattggaactattccagagcctcattcgattatctgtaccaacagtgaggaggtgaagtccatcacttgtaaaacataagccattaactttcccattatgagcagtgtttgctgattcaacagcttgtgactttttcccattatgttgatcaagagtaatcaaacatcctgatgctcttctcacatcccataattttactctactgtcagcacttgctgttgccaagatatagtcataacgtggagaccaggaaactgctaatatttcttgtctgtgaccctgtagaatgtgagaacaggatccagacttcaagtcacaaagttgtactttgggtcctctagtaccaactgctaccaaacagtgcttggtggagactggagacatatgatgactataaactgtttcctcaaaattaaatacatctgcagtttgtaatgtatttgtatcccatactttcagagttttatcaaatgagcttgatgtgaacatgccagtgtcatgaggataccactgtacagtctccacactgtatctgtgaacatcaggatgatctctgccaatggaacacactgctttacatgtgtaataagattgtctgctggagttctcaaggtcataaagtacaatcacaccatctgaaccacctgataacatgtatctcccttcaacaggttcaatgtcaagggtgttaattccaccgccgtggattctttcaacatctctgtctttatttaattccagtcccaaaactctccgtgttgactctgctctccgaaggcgaagagggtcctccaaacccgtttggcgtgcggacaaaaaccccagcatatcgtgtcctcacaccggctggagcactggacgtcgccatgacagagctcaggggcgggact

SEQ ID NO: 18840 - RNA, 7259 nt, Homo sapiens
  source 1..7259: mol_type = other RNA
tgcaaaagtaattgcagtttttgtgattacttttaataaaaacaaaaaacaagaagccacatggcagcaaaagaagtatgccttctgtatctgaggatgttgctgatagagctagcaagatagaaaaatttgtattataataaatgatttgtaataattctaagcacccaggaggtttacaacagtgattctaggtagcacattaagaactacacacatattctttgcaaagaagaaaaaatgtttatgattaaacttcgttagttttcttccctgaatttaatacttttccagaattaaaacagaagaactagcactatcctgagccctagatttaaccttccgatgtccagaaattcattacaatagaaagcaaagtgattgttttcctttctgtaattagctttccctgctatatttttcgacaggcaatattctaattgtgctaggcttgccattccatttctggcatagttagagtgattttaagtttactgctttagtgataagttttttagttcgggctcaataattagcacctgaacatggaaaacattaaattaaaaaaatggaaatttaccaaagtatttgtttataaaaattatagaattcacagaaacgtctttagcttctctagtcttcagtagttatatcatttttatagaaataacaaagtattagtatattactcaacagtaatgaaatatttctgaatgaaaactgtgtagcccttatttaagtacctaatttgaggttttcctttccattgtgaaatagtgattttgctttgaaaaataattgagattagtttgctgatgcaatatttttctaccactgtctcatttcgattttaaataataaagctaatggtgtgtctctcaccaatactgagctctacaaacctatgtgtctcttactgaagagcttcgttttgaaattactttatctattattataattggtacagtttaaggttttgtctttagagaattttttaaaggttttaaaatctattttaaatggggctttttagtataaactggacacaaggaacacttcagttcatgggataactttttttctctattaaggtgttcccttaattctaaagtaaaggcatggtagcaagtttaaaagagaggtcaagctgatctacgatgtgattttttaggcttctggttaaaaatagatttatggctatgttaataaaatgtgcatttattatttctacatatttttttaaaactaggcatttcataggtgtaccataatgactagttaaaaatggaatcaaagtgaagtgaacaaatggcctaagtattctttgaaatatggcagaatataagtaccttaggtgacgaaaggacagccaagacagcgtgaaaggaaaacatataaaatgtacaaggcactggagagaagttatacatgatcgctgccttcataatagattcattgatatacaatgtgaataagggttgacaaataccagttgaataaacaattattaaaaagtttcaagtggaagcctcccatatttctccactatatttttgcaagtgcttaacaaaacaaaacaaaacaaaacaagggtttagggtggggaggggaataaaacaataatcaaaagtctcccctaattatcacagtcaggcctgaattagtaaccttgaatatcaaacacaaactctcaaagtataggacagaaacaacaaaacaagtaattattaagcacctactacatgccaactacagttctaagaattgaaacaaaacaaaacaaaaagggcaaggagaaacgaaaagataagacaatgaaagagaagtcgaagtcaggcccggcacggtggctcacgcctgtaaatcccagcactttgggaggccgaggctggtggatcactagagcccaggagttcaagaccagcctggccaacatggtgaaaccccacctctgctaaaaaaaaaaaaaaaaaaaaaaaaaaaaaattagccaggcgtggtggtgggcacctgtaatcccagctgcttgggaggctgaggcaggaaaattgcttgaacctgggaagcggaggttgcagtgagctgagatggcgccactgccctctagtctgggtgacagaatgagattttgtctcaaaaaaaaaaaagggaagaaaggaagaaacatagagaggtcagttacatgcaatttttagataatccaaaaaagaagaaggaaaaaggagaagcaacaattagacaaatattagaagaaaatatacctgagctgagaaaaggtttggaccttcattgaaagagctcccaagaagtctaagaagtgacggaagagaataaaaaaagacatcagatttcttgacgagattaagaaactgtaagtttttacttttttcttttaaacctcagtttacaagcttccagctgtaacgaatgaattccctacaaagggaaaaaaaaccaaagtggctttggaattctcaactgcaataccagaagctagaaaaaagtgggcacaatatctatagaccaacaaaacaaaaggactacaacccaaaaatcgtatacccagctaaactatcatttcagaggggaaaaaaaagatgatattcaacaactaaattgtacaaattgtacaccaaaatataccaagaaaaatatagtacagttccaagtcttcactaataaacatgtagccttgaacaggggaccagctgaaaacaactgggggacattcacaaaatgcagtatgatgcagttaacaaaaagaataactttgttataacaaatgacagagagggatttatataagctgtaactgcaaaatataatttaaaaactttgtatatcccagttctgcaaaataaaaatacatcccctatatgtctgcatagatatatataggattgcaatatgaaagaacacagtctaggttaataacttggtttgtggcagcaggggtaaggactggggaatgtggtactaatgtggaaagagaggggtgtttataacaacagcttgttgaacatcccattatgtaaaattatatgtatcataagagattcatgaagaatgaccatgaaaatgttagtggtggttaccttatggtattataattccaggtgaccactaccttcctttttagatttttatgttgtttgaattatttataatgagcctatatatctatataactagaagtaagtaaaacagttacttgcagtttggaagcagacttcctttttcttaaaaataaatttccaattttaatagcttttcttttctttttcttttgggagacacaaggtctcgccatgtcacccaggctggagtgtagtgacacgatcttggctcaatgcagccgtgactttacaggttcaagtgattccccagcctgagtctcccaagtagctgggactacaggtgtgcacaacacacttggttaatttttgtattttttatttagagacgaggttttgccatgttgcccaggctggtcttgaactcctgagctcaagtgatctgcctgtctcagctcacaaagtgttaggattacaaccaccgtgcccggccaatagctttttcaaactagctttttcaaaggtcaaatgcatcctcaccaaggggacaagattgaaagtagaatggcctgggcttaataaatcaatgatttgaaactatcagaagaaaacatggagaaaatgctccatgacattggtctgggcaatgatttttttggatacgatctcaaaagcacagtaacaaaagcacaagtacagaaatgaaattacatgaaactaaaaagcttctgcacagcaaaggaaacaattaatagggtgaagagacaacctacagaatggagaaaaaatattaactatagatctgatagggggttaatatccaaaatacataaggaactcaatagcaggaaaacaacccatttaaaaatgggcaaagaacctgaaaagacagttctcaaaagaagacatgcaaatggccagcagatatatgaaaaaattatcaacatcagcagtcaccagggaaatgcaaattaaaacaacgagataccacctaacacctgttagaatggctactatcaataacacaaaagataacaagtgttggcaaggatgtgaagaaaaaggatttcttgcattattgtgaagaaaaaggaattcttgcatattcttggtaggaatgtaaattagtacagccattatggaagacagtatggagtttctgcaaaaagttaaaaatagaactacatatgatccagcaatcctaatactgggcttatatccaaaggatatgaaatcagtatgtcaaagagatatctgcactaccaggttcactgcagcattattcacaatagccaggatatggtatcaacctaagcatctgtcaatggttgaatggataaagaaaatgtagtacatatacacaaacagctgatctcatagaagtagagagtagaatggtggttaccaggagctagggttgttggagaaacattggtcaaaggatacaaaatttcagttaaaaagggggaattagtgcaagagacctattgcacaacatagtaactatagttacaattacaagattactattaattttgaaaaataagagaatggatgtaaagtgttcttaccacaaaatggtaaccatgtgaggcatatgtcagttagctagatttagtcattctataatgtatatatgcttcaaaacagtatgttgtacatggtaaatacatacaattttatctgccaattggaaaaaaaaatcaattgtaaaagcaagtgtttggaaaacatttagctggaaaggtctgataggaggtctaacccttatacacttaaaaactcaacaactggctgggtgcagtggctcaagcttataattccagcactttgagaggccgaggcgggtggatcatttgaggtcagcagttcgcaaccagcctggccaacatggtgaaaccccatctctactgaaaatacaaaaaaattaaccgggcgcagtggcgggagcctgtaatcccagctactcaggaggcttaggcaggagaattgcttgaacctgggaggtgaaggttgcagtgagctgagatcaaaacactgcactccggcctgagcgacagagtgaaactccatctcaggaaaaaaacaaaaaaacaaaaaaccctcaacaactgtttacttttggtattcaagctcataaaagcctcatttactagtctactgctggtaaggatcaggaagggaaaattaagattaccttcatgataatcacgtgtgggttgacacagacggagacaataacatagaaattttattacagcatttcatgtttaagccagattccctgccaggatattttctgcttgaattaatgaggcaggatttggtcataccttaatgagtttcacagaaaaagagttcaagcattagcgcaaactgccttctgacattaaaataaaataaagcaaacatgggattttcacaaagttaaaagcctcctgtgatgcacattttggatagtaggagacattgagccccaaaatgtttaacataaagcatggttaattaaatgaaaccactgaaaaatgtgaatacatgaagaagaaagaataaaataattttgatgttaccatttcaactactatttttgatataatcattcttggcaaaatcattcttaaaggtggaaacgagcaggctgatagtacagcaagtaagagaaagtcaatactgatggcctccacttgctgatcctctgagactgcatcttatagttcataaaatctgctgaaggtcacaactgaggtacaacgacttgtgttacttgtactgtagcaatgagggctttcccaggccacaacatctgggatcaaggaacacattttgactaaataaactatacagaagtctgttttaggattttatgcaaatattaacctcattttaaaacatgaggaaaaatattacccacatttagggctaatttagctgtcaggaatagaccatacagttgaaaaaaacacagtctcatttaaaaagtttcagcagagacaaaaaggtactaaagatgatattcatccttcttcatcactgctgctccaggcatcttcaaaggccggatttaattgtgattttgttgtagtctcatcatcatcaggaactggttcatataaggatggaacccaagccagaatgttgcagtctctgctaccactataaagttcctggaaatttgactgaaatacacagcagtcaacagttttataatgtcccttaagcatagttatctgttctcctgagtaaactgtataaacagcaatggtgctaccatatggtacaaaaacaaattctgaactgcagccacaggagacagtgaatttcaatccttttttactgttattacaaacttttccatagttcacaagtgtgttttctccattggaactattccagagcctcattcgattatctgtaccaacagtgaggaggtgaagtccatcacttgtaaaacataagccattaactttcccattatgagcagtgtttgctgattcaacagcttgtgactttttcccattatgttgatcaagagtaatcaaacatcctgatgctcttctcacatcccataattttactctactgtcagcacttgctgttgccaagatatagtcataacgtggagaccaggaaactgctaatatttcttgtctgtgaccctgtagaatgtgagaacaggatccagacttcaagtcacaaagttgtactttgggtcctctagtaccaattgtaatgtatttgtatcccatactttcagagttttatcaaatgagcttgatgtgaacatgccagtgtcatgaggataccactgtacagtctccacactgtatctgtgaacatcaggatgatctctgccaatggaacacactgctttacatgtgtaataagattgtctgctggagttctcaaggtcataaagtacaatcacaccatctgaaccacctgataacatgtatctcccttcaacaggttcaatgtcaagggtgttaattccaccgccgtggattctttcaacatctctgtctttatttaattccagtcccaaaactctccgtgttgactctgctctccgaaggcgaagagggtcctccaaacccgtttggcgtgcggacaaaaaccccagcatatcgtgtcctcacaccggctggagcactggacgtcgccatgacagagctcaggggcgggact

SEQ ID NO: 18841 - RNA, 77 nt, Homo sapiens
  source 1..77: mol_type = other RNA
tgcaaaagtaattgcagtttttgttttctttggctcaagagtgaaattctgaagcaggtgatgacttgaaataggtc

SEQ ID NO: 18842 - RNA, 1962 nt, Homo sapiens
  source 1..1962: mol_type = other RNA
tgcagctctggtggaaaatggaggacatgtccagcaaggtgctccgctcatccagggctgccgcaaacgccttccactcctgctccagctgactcgcgatctgcctgatctgctgcgaggcatagtggccagactccaccagacgattggccaccgacatgatgcggtttatatttacatacacgttcatacagttcatggcaaagtgattgtgctgcgtctgaagctccatggcatgagggtggctggtcccaatctctgtgtagctgtttagaaacaggcctttgttgtgtgtgatccagtcaaacatcttctcagcatcctgttcaaacagcctcagctggaagcactggtccagcttcagcttcctcacatgccacatctggtgcagatgctgccgtgtcgagtgcagccggtccagcatggtggacaccttgggcaagaggttctgcaggtccgcattgcctgagcctgagttctttttgggaaagctttcactgctctgtatcctctgaagcagcttctgtccctccaaatccaggtcctcgatgggggccttaatcaccttcttcttcagctgagaatgttcctcgatcatattccgagccccctctaaatcctgaggcagctccttcttagctaggatgtcctgaagttcctccagccgagacagcatgtgggtggcattgctaatgtagtcttcaaaagcaactctgatttcaatccattcttcgtggttgtattccaggcagccatcaaactcaggagttagctgagaaggatcaactactttggtaaggccttctaaagagaccatatttgtctcaaattcaaatttagaactgccaaaattagtcctctgtttctgccagaagttgtctggcttgatgatcagggccacatggatgcagcaggggaaggactcctgcaggatcttcagaaggggcttgatggagtcccacttggacccacgcatgtccacgatcaccgtgaagccacgcttgcagacctcctcgctgggaatacaggctagataggaaatgagtctcctgagatcctcctgtcgtattctgtcatgattgctgcgggccggaaacgttaaaatgggacctccacgtttatctctcccacctgaaaggtatgcaactttttccttcaaaattggtaaaacatccatagctttcatttcatcgttttttcgaaaccatgtccacactgcacgccatctgattctctccaagtaggaagggcaagaggaacggcagcctcgtgctgccctaccaagcccgcgccttaacatctctgcgatgttagaagtcaccaagtctgatcaactggggcttcaggattcttacctggaaacagggaaaagtgggagggagaggaggtgcccctcagagaattgttacaaggtttaaaacttcacatgtatttcttaaaaggtggtcccataaacacctgcatcagaatcctgtggaacagttactcaaaatgcaggttccaaagccccgccccaaagatactgagaaaagaggtctggaaggggctgcattttactgtttccaagacaatgcttaggtcaggttaaaagcttcccagcttcttttattcttagtgtttgtctcagagcagatgatttactggctgggggtctgagctaaggattcaaaacaatacaaaatgaggttgcgatgaaagggaactaagacatcatctaacctactgggtttcaaacttttgtgaccttaacccacattaagaaataccttttacaatacaactcaatatgcttgtgggtttggttccagacaactgcaataaagcgagtcacacaactttcttggtttcctagtgcatataaaaattatgtttacactatacgttacatggtacatttatcctatactgtagtttattaaatgtgtggtagtatttgtctttaaaaatgaacacaccttaatt

SEQ ID NO: 18843 - RNA, 1498 nt, Homo sapiens
  source 1..1498: mol_type = other RNA
tgcagctctggtggaaaatggaggacatgtccagcaaggtgctccgctcatccagggctgccgcaaacgccttccactcctgctccagctgactcgcgatctgcctgatctgctgcgaggcatagtggccagactccaccagacgattggccaccgacatgatgcggtttatatttacatacacgttcatacagttcatggcaaagtgattgtgctgcgtctgaagctccatggcatgagggtggctggtcccaatctctgtgtagctgtttagaaacaggcctttgttgtgtgtgatccagtcaaacatcttctcagcatcctgttcaaacagcctcagctggaagcactggtccagcttcagcttcctcacatgccacatctggtgcagatgctgccgtgtcgagtgcagccggtccagcatggtggacaccttgggcaagaggttctgcaggtccgcattgcctgagcctgagttctttttgggaaagctttcactgctctgtatcctctgaagcagcttctgtccctccaaatccaggtcctcgatgggggccttaatcaccttcttcttcagctgagaatgttcctcgatcatattccgagccccctctaaatcctgaggcagctccttcttagctaggatgtcctgaagttcctccagccgagacagcatgtgggtggcattgctaatgtagtcttcaaaagcaactctgatttcaatccattcttcgtggttgtattccaggcagccatcaaactcaggagttagctgagaaggatcaactactttggtaaggccttctaaagagaccatatttgtctcaaattcaaatttagaactgccaaaattagtcctctgtttctgccagaagttgtctggcttgatgatcagggccacatggatgcagcaggggaaggactcctgcaggatcttcagaaggggcttgatggagtcccacttggacccacgcatgtccacgatcaccgtgaagccacgcttgcagacctcctcgctgggaatacaggctagataggaaatgagtctcctgagatcctcctgtcgtattctgtcatgattgctgcgggccggaaacgttaaaatgggacctccacgtttatctctcccacctgaaaggtatgcaactttttccttcaaaattggtaaaacatccatagctttcatttcatcgttttttcgaaacccgcgcctcccggtcctccgagcttcagctcggccaccgtccccactccctgggcagtgagtgccgtgactgccccgtttcacagaagtgtagaccaaggccggggagatgacaggctagagggccaagcaaagaaacccggctgctaatggggtcgaggagggtccaggtacaaatcagccagagacaggcacagatcaaagaccaatttcccgtcccggaccggccccggctcagtccgctcggcctccggggtaagagcctccgcccacgccatctccgccgccgcctcc

SEQ ID NO: 18844 - RNA, 1739 nt, Homo sapiens
  source 1..1739: mol_type = other RNA
tgcagctctggtggaaaatggaggacatgtccagcaaggtgctccgctcatccagggctgccgcaaacgccttccactcctgctccagctgactcgcgatctgcctgatctgctgcgaggcatagtggccagactccaccagacgattggccaccgacatgatgcggtttatatttacatacacgttcatacagttcatggcaaagtgattgtgctgcgtctgaagctccatggcatgagggtggctggtcccaatctctgtgtagctgtttagaaacaggcctttgttgtgtgtgatccagtcaaacatcttctcagcatcctgttcaaacagcctcagctggaagcactggtccagcttcagcttcctcacatgccacatctggtgcagatgctgccgtgtcgagtgcagccggtccagcatggtggacaccttgggcaagaggttctgcaggtccgcattgcctgagcctgagttctttttgggaaagctttcactgctctgtatcctctgaagcagcttctgtccctccaaatccaggtcctcgatgggggccttaatcaccttcttcttcagctgagaatgttcctcgatcatattccgagccccctctaaatcctgaggcagctccttcttagctaggatgtcctgaagttcctccagccgagacagcatgtgggtggcattgctaatgtagtcttcaaaagcaactctgatttcaatccattcttcgtggttgtattccaggcagccatcaaactcaggagttagctgagaaggatcaactactttggtaaggccttctaaagagaccatatttgtctcaaattcaaatttagaactgccaaaattagtcctctgtttctgccagaagttgtctggcttgatgatcagggccacatggatgcagcaggggaaggactcctgcaggatcttcagaaggggcttgatggagtcccacttggacccacgcatgtccacgatcaccgtgaagccacgcttgcagacctcctcgctgggaatacaggctagataggaaatgagtctcctgagatcctcctgtcgtattctgtcatgattgctgcgggccggaaacgttaaaatgggacctccacgtttatctctcccacctgaaaggtatgcaactttttccttcaaaattggtaaaacatccatagctttcatttcatcgttttttcgaaacccggatcggaagaaggccgcgatgtcggccaggtccttggccgcctcctctgccccctcgccggcaccgcccccgcagcccgagccagccgcgctggccgccgcggcggggccggaggacgcggcgggggcggcggctccgccgctgctgccgctcatggctgcggcggcgcccgcggccgcgcccgcctcgggccccgcgcccctagcgccgcgtgccgcccgctccgcgccgggcctggcggcgccgagcacccagctgcccgcgcccggcgcgcggacgcagagccccggggcggcggggggcggcggcggcggctcggcccaaggagcgcgcccacatagacgaggactccgcccggtagccgcgagctggccgaggggcggaggcgcggagccacggcctcccgggcgccggccggagcgcgggcagcagcacgcgcctcccggacgcgcagtcgcgagggcgggggcccgtggccggcgagacctccgggatcacgggcgccggcggctgccgcgagcctccatcttg

SEQ ID NO: 18845 - RNA, 1747 nt, Homo sapiens
  source 1..1747: mol_type = other RNA
tgcagctctggtggaaaatggaggacatgtccagcaaggtgctccgctcatccagggctgccgcaaacgccttccactcctgctccagctgactcgcgatctgcctgatctgctgcgaggcatagtggccagactccaccagacgattggccaccgacatgatgcggtttatatttacatacacgttcatacagttcatggcaaagtgattgtgctgcgtctgaagctccatggcatgagggtggctggtcccaatctctgtgtagctgtttagaaacaggcctttgttgtgtgtgatccagtcaaacatcttctcagcatcctgttcaaacagcctcagctggaagcactggtccagcttcagcttcctcacatgccacatctggtgcagatgctgccgtgtcgagtgcagccggtccagcatggtggacaccttgggcaagaggttctgcaggtccgcattgcctgagcctgagttctttttgggaaagctttcactgctctgtatcctctgaagcagcttctgtccctccaaatccaggtcctcgatgggggccttaatcaccttcttcttcagctgagaatgttcctcgatcatattccgagccccctctaaatcctgaggcagctccttcttagctaggatgtcctgaagttcctccagccgagacagcatgtgggtggcattgctaatgtagtcttcaaaagcaactctgatttcaatccattcttcgtggttgtattccaggcagccatcaaactcaggagttagctgagaaggatcaactactttggtaaggccttctaaagagaccatatttgtctcaaattcaaatttagaactgccaaaattagtcctctgtttctgccagaagttgtctggcttgatgatcagggccacatggatgcagcaggggaaggactcctgcaggatcttcagaaggggcttgatggagtcccacttggacccacgcatgtccacgatcaccgtgaagccacgcttgcagacctcctcgctgggaatacaggctagataggaaatgagtctcctgagatcctcctgtcgtattctgtcatgattgctgcgggccggaaacgttaaaatgggacctccacgtttatctctcccacctgaaaggtatgcaactttttccttcaaaattggtaaaacatccatagctttcatttcatcgttttttcgaaacccggatcggaagaaggccgcgatgtcggccaggtccttggccgcctcctctgccccctcgccggcaccgcccccgcagcccgagccagccgcgctggccgccgcggcggggccggaggacgcggcgggggcggcggctccgccgctgctgccgctcatggctgcggcggcgcccgcggccgcgcccgcctcgggccccgcgcccctagcgccgcgtgccgcccgctccgcgccgggcctggcggcgccgagcacccagctgcccgcgcccggcgcgcggacgcagagccccggggcggcggggggcggcggcggcggctcggcccaaggagcgcgcccacatagacgaggactccgcccggtagccgcgagctggccgaggggcggaggcgcggagccacggcctcccgggcgccggccggagcgcgggcagcagcacgcgcctcccggacgcgcagtcgcgagggcgggggcccgtggccggcgagacctccgggatcacgggcgccggcggctgccgcgagcctccatcttgatttcaat

SEQ ID NO: 18846 - RNA, 1261 nt, Homo sapiens
  source 1..1261: mol_type = other RNA
tgcagctctggtggaaaatggaggacatgtccagcaaggtgctccgctcatccagggctgccgcaaacgccttccactcctgctccagctgactcgcgatctgcctgatctgctgcgaggcatagtggccagactccaccagacgattggccaccgacatgatgcggtttatatttacatacacgttcatacagttcatggcaaagtgattgtgctgcgtctgaagctccatggcatgagggtggctggtcccaatctctgtgtagctgtttagaaacaggcctttgttgtgtgtgatccagtcaaacatcttctcagcatcctgttcaaacagcctcagctggaagcactggtccagcttcagcttcctcacatgccacatctggtgcagatgctgccgtgtcgagtgcagccggtccagcatggtggacaccttgggcaagaggttctgcaggtccgcattgcctgagcctgagttctttttgggaaagctttcactgctctgtatcctctgaagcagcttctgtccctccaaatccaggtcctcgatgggggccttaatcaccttcttcttcagctgagaatgttcctcgatcatattccgagccccctctaaatcctgaggcagctccttcttagctaggatgtcctgaagttcctccagccgagacagcatgtgggtggcattgctaatgtagtcttcaaaagcaactctgatttcaatccattcttcgtggttgtattccaggcagccatcaaactcaggagttagctgagaaggatcaactactttggtaaggccttctaaagagaccatatttgtctcaaattcaaatttagaactgccaaaattagtcctctgtttctgccagaagttgtctggcttgatgatcagggccacatggatgcagcaggggaaggactcctgcaggatcttcagaaggggcttgatggagtcccacttggacccacgcatgtccacgatcaccgtgaagccacgcttgcagacctcctcgctgggaatacaggctagataggaaatgagtctcctgagatcctcctgtcgtattctgtcatgattgctgcgggccggaaacgttaaaatgggacctccacgtttatctctcccacctgaaaggtatgcaactttttccttcaaaattggtaaaacatccatagctttcatttcatcgttttttcgaaaccctggcccgccctcctccgctctccaacccggagtctgcatcctccctgccccgtg

SEQ ID NO: 18847 - RNA, 8587 nt, Homo sapiens
  source 1..8587: mol_type = other RNA
tgcagctctggtggaaaatggaggacatgtccagcaaggtgctccgctcatccagggctgccgcaaacgccttccactcctgctccagctgactcgcgatctgcctgatctgctgcgaggcatagtggccagactccaccagacgattggccaccgacatgatgcggtttatatttacatacacgttcatacagttcatggcaaagtgattgtgctgcgtctgaagctccatggcatgagggtggctggtcccaatctctgtgtagctgtttagaaacaggcctttgttgtgtgtgatccagtcaaacatcttctcagcatcctgttcaaacagcctcagctggaagcactggtccagcttcagcttcctcacatgccacatctggtgcagatgctgccgtgtcgagtgcagccggtccagcatggtggacaccttgggcaagaggttctgcaggtccgcattgcctgagcctgagttctttttgggaaagctttcactgctctgtatcctctgaagcagcttctgtccctccaaatccaggtcctcgatgggggccttaatcaccttcttcttcagctgagaatgttcctcgatcatattccgagccccctctaaatcctgaggcagctccttcttagctaggatgtcctgaagttcctccagccgagacagcatgtgggtggcattgctaatgtagtcttcaaaagcaactctgatttcaatccattcttcgtggttgtattccaggcagccatcaaactcaggagttagctgagaaggatcaactactttggtaaggccttctaaagagaccatatttgtctcaaattcaaatttagaactgccaaaattagtcctctgtttctgccagaagttgtctggcttgatgatcagggccacatggatgcagcaggggaaggactcctgcaggatcttcagaaggggcttgatggagtcccacttggacccacgcatgtccacgatcaccgtgaagccacgcttgcagacctcctcgctgggaatacaggctagataggaaatgagtctcctgagatcctcctgtcgtattctgtcatgattgctgcgggccggaaacgttaaaatgggacctccacgtttatctctcccacctgaaaggtatgcaactttttccttcaaaattggtaaaacatccatagctttcatttcatcgttttttcgaaacccttctgccatgtcctcttgggtaatttattaatcttttttaaaaaacggttaccacgaaaataaaatcgaagtaaaacagtcactatctgccaaaggttaacagttggcagtgtccctcaggatcccagaacaccaacaaacaacctctagatatcccaaatgggcagtgaggagcagccagcatgctgtaactgcggccgcatgccttccctcctcagcaaacgggaggggcagaaacagcacagaaagttttgttccagtttttgatccaagtctgaaaccaaacccattatggagggggaaaaaaatgagactctgatggttaaatagcaatgttaaattcttttctgtttttttctctttttaattactcagagtttctttagggcttttcttgggggggaagggaggagtttattgttttcaattttagtcaaagaaagtaatactttatttgtttacatttttaggggatgcaataattattctgaaagagtactttaacaaactgatcccttttaagcatcttttaaagcaacaagtctccaaggacatattttttcattatgtaaacatacatatgtttactgcatacttactattaaaggaaggggagagaaaagcccctgcttacatcacaatcttgctgatggagagaagtcacaaaaaaatgactcccaagggcacaacatacgtcccacagaactgcagttcagagactttcaacggaggggagcaagggaaagcctcactaaggttgtagcttctgtaaaagtccaggccaccgggaacaaacctagctgtgataaggagttagccccaggaggccagaaggaacaggcatccttctgaaccctaacgaagaccccacctccccagctcatggagcagctggccccatcctagagatgcactgttgtctacctggtgctgcccagaggcctgcggaaaaggatggggccctggcccagctcagaggaaagggagcacaaaggatgatgcgctacagccaggcctgcaggcaggggcacgcaaatgcctgtagctgccacccttgctctagaacaaagtgcacggcaaagtggaggggggggggtctccactgtatttggtccaattttccttaggaaatctctggaaaatcagggaaggatttttaaaaatcatcagaactccaaattcatacctagggagcacttcacctgtcaggagaaattaagggaattcttaaaggctagtgaatgttccaacagataatgtcttagaaagaaaagcaaatcatgagatttaatcagagaaaaagtacagcaagtgtaataattaatggcattttcttacagaccaagctcctacatgtaaatttctcactaatttttaacactttaattatcaacaaaattaaggcatagaattgatactgtcattgaatcatgtatgtattaccacaagatttttagctatgtctatggacaagaagaaacttgcattgtatttgataaggcaatcatttctaaaactttgctattccacctacactctgacaacaatttctatcagatataaatttgtcccaaggtagaagcatctctaaagagtgagccaaagactaacattaagatccagggaaccaagatgctttctcagctaagagggaaccaacaaggagtaataggcggttctaccaaataggaggacgtgcactctctctccctgagcctcacagcagagccggggtccttcccacttcccagaggagcctgctcctgaggaataacacagagaagtctcgtttatcaaatcttcaggccacacagctcagagacgtcattactgtgttggatgaaaagaaaaaaaaaaaatgcccttcaaagatttgaacaggaagaaccaaaagtaataacatgaaattcaatgatatgtgggaagtggtgttcatattcaaaatattaatttcttaaatacaagtcagggaggatggggatggggagaaggagattaaaaacagaggactgaatattctggagagttctatgaggtcagacctagaatttcagacccacatcagcccggagtgtagaaactaccagaaaaggaatagtgagggcaagtggggatgcaaaagagcccaggccgggaggggcgtggccaccatgtggtcttcagactttctcttctttctcctgccatccattcaagactctgaacttggcctcaatcctctaatccacctttacagacccctgacattggtctctaagtcaagcagggggcagccagcgttttcaggacactgaaatggccctcaaaggatttctgcagtgcagctgcctgggggcaaccgtagacacaggtcctgtgtgagtggtcccacgtgccatctcacagactacgccccccagaaacgctccacatccactcacaggcctgcccacgaccatctgcaatctggcacaaaggccatcacagattctgagattgggcaggccacagaatggctgtgaagttctaacagacagtgccagggaccccccaggcaggaaacaacagatgacggtgacagataactagttctacagatttgtctgggctcgggtgaagcagcccacaacaattttagtttcaacaaacaccaaaaacttcagagaagtactaacaaaatttcaagcaggccagtatctgaaaggacatttccttttcatggttctctaatacactttaaggcatccaagaataatacggtatttgtagaaattctatatcccttaaataagatgtcttttttttttaagtctgcagtgttagctgtatgtcctacaaaaaggtaagagcctaagaaatacagctaatagaagaatgaaacaaaaaaaaatacattgtagtattccattgttatttttttataatccatataatggaaacaaggaaaattctaaatgtgaatgtttatgaacacaattttcttgcatgttctttataccttaacttttttctgaaggatttccctagacaaaattaaatattttagtatatacagaaaataagccaactcaaatcataaatttcaaaagaaaattaaaactgcctacctacctatatttcttttttttttttgtgggggcactggggggacatgggaccactcactctgtcacccaggctgaagtacagtgatgaaatcagagctcattgcagcttcaaactcctgggctcaagagatcctcctgcctcagcctcctgagtagctaggactgcaactgcgtgccaccacacccagctttttatttttttgtagagataggatcttgctatgttgcccagactagtctcaaattcctggcctcaagcgatcttcccacctcggcctctcaacttgctgggatgacaggcatgagccattgtgtctggcctatattttcatatgcaaagatcagacacttctaacaacatggtctgccttttttatttaagttaaaaatgtgattcttacaaaggaacaatttaggttatattctttagaaggcaaacaatccttatttatttaagaatactaacagctttcatttcaaacaatactaagtctcagcatagttttataaaaagttgtaaagtcagttatcttcttttgtcccattaccttcaaaataatcttttttaatccaatgagaataggaagctccaggcaacatctaatgatcggtttggaaattcaggccacagactgaaaatatcagcatgtaaccagcttttgatccaggtaactttaagaggttgtgccagaaaactagggaatataacgcataggctttaccacatctatattacagttaatcttttttttttttttttttttttttttttgagcaggagtcctgctctgtcacccaagctggagtgcagtggtgcgatctcagctcactgcaacctccgcctcctgggttcaagcgattctccagcctcagcctcccgagtggctgggattataggcgcgtgccaccacgcccagctaatgattttgtatttttttagtagagacgaggtttctactggtcatgttggccaggctggtctcaaactcccaacctcaggtgatccacccacctcagcctcccagagtgccgggattacacacctgagccaccatgcccagacagttaatcattaatttagccaatacatgttcaaaaatcaaatgaacttaaaatatgtgtaaaattccagattgaggctgggtgtggtggctcatgcctataattccagcacgctgggaggatggcttgagcccaggagttcgagatcagcctgggcaaaacagtgaaactgcactgctaccaaaagaaaaaaaaaaaatcaaaaactgagctgggcttcgtgatgcatgcctggctgaggcaggaggatcacttcagcggagctcaaggctgcagtgagccgtgattgtgccactgctccaaattgggcaacagagtgagaccctaaaaaaaatccagattttaagaaaaaaaaaaaaaagctttgttgatttatttaaatatttatattactgaagaattctgagggcagaacaagtgaaaagaatacatttttattttaaaatggttttaaaattgtaatgtagtattacagagtaattaagaacaaatacaaaacaattcctctaacttcaccgtatgtttgagtctagcacatggtaaagaagtcacagggtacctaactgctaaacaggatttctctctccattctgagacaccagacccacaaaggtggggggtggggccaaagcggggtgggtggcaggacgggacaccgacgtgctggccgggagcagcaggggactatgaccaaaactcttccctcactccaaatgggaaggcggtgacaaaggctttctcaccaccctccagtcccggcttctgcgggggtggggggagtacaaagacccccttctgagctcttggtaaagaagggtaggacgcaagccaggtcctgggggctgacaaatcctgattcatggctcaagtcacacttagctcacacacaaaatgagcgattcagccactccaggctatggggaggaggcttcttcaaatgtgctgtaggtctgttttcaaacagaccaccactgacaggaggtgctgactcagcagcacccctgtgaccactctccttggccaactgtccatgcctttatgtatcctggactgagtcaaacatcattttatccaagttaggggtgagccacaaaaaatgaccagtgggagtcataaatatcttcacatgactctcaccctctacatactgaattatgaaactatggtcagtcagtaggtcgagtcatcacacatcctagcttgacagacacagtctcagtttacccctactgttctagaataattattggtaacaccctctttcactctcaacaccatctctgtttagacaattacgcggtcagcttatcaagaaatgtgaagatatcaaagcatcaatatttgacagcaacacctgtcacctttctaataccaggcaggcacaaggctttttatccacaccataagagggttcctaacatgcggccagaacacaagattaacagcctacgtctctcacatggaatctgtgcaaacatctctatgccagtaaatttgaatattattcattttctccccttttttaattgacagcattcctgtgtcaacaaccatcacctacaaatgacctctcttaaaaatccttgtggtgtaggaccacacgtacaactctgtttctgctgcttgtttggcaaatccaaagtaataaaggccgaatggaatctctgccctagcagactatttttagggaagaatggttaaaagaagtggcaaaatgaattactccacaaacaaggaaaaccatgaatacaagagtatttgttaaaagcaaacacaaaagccaaacacatgacaaacagtatctgtaatattaaattaaatggtgaataaatataaaataatcaagtaaaacaaaaaagtagacaatgttgataaaatacttgcagtgcattagaaacagagccaagccacggtatggtgaggaccgattttgcttttctgtttaataatgggcctgtgaaaattccagagaaagtcttgcattagcatgaagatgcaaagcagcccctccttcctgcagtccatatactcagccctcaagacaggcagaagggaaactcctaggcacccaagcccagggactgatgagaagtgggagacctctgggcaggagacaggaggagtggttcttcctctccaaggggtcctgggctctgggacccagcgagggatggaagccagtcagcccggcaatattctctctctaccctgttagctttttttgttgttgttgttcttaaatttcctatctgatcataaaccacaggtagcaggcttaaaagtacaagaatcctgggctatccttgaagacacccaggttccagaacaggagctccagcaaggatggtacaaacctaggatggtgcgtttcagagcagtcagataccaagaattatcatgaaattcacacaagtgccagaagtgcatgtcactaaaaagacctctatgtttgaaaatccccataagaagattttcataacatctgctcatatcccggtgattaccaaaaaaaatttaaaagtgccctttaaacttgtgaaatataagccactaaaagcaaaacttaaaagtggtggcttgtaagagttttctcacgtatataacataaataataatctgttttcaacactcaagtgaattccagaataaatcacctgccctcctggggcataactgtatgctcaccactgtcaacccatgagtgccctgggcgctcaaacctcagggcagagtccatggaacccaattacagtatgtaaagctggacacacagtgtttgaaaacaggttgtttgtgcttacctaagaatattcttataaaaactaaatgtaatggtcaagtgtttcatttctaaaatgaatctattataatattatcaaccctgtaatatgtgcataaaatatttaatggccataaagaaaagttaaaaccagattttcaagtgcctgtgacttaagaaaaattaaatgttttggctctttccatttacttaacagtaagcaaaaaatgttacttttgaaaagttcatgtttctaaattttaaaatcatctttaaaagaatgaactgaggctgggcatggtggctcccgcctctaatcccagcactttgggaggccaagtgggtaggagttcaagaccggccaaggcaacttggttggtgaaactccaccgctacaaaaaaatacaaaaattagtcaggtgtggtggcacacggctgcaatcccaggtactc

SEQ ID NO: 18848 - RNA, 2058 nt, Homo sapiens
  source 1..2058: mol_type = other RNA
tgcaggggtcgggtgggccaggggtcccccagcacctcgccaaagcttcctgggcctctctggctctcccacaggcaatgccaaggctgcgggtgggtatcgggcgcccggcgcaccctgaggcggttcaggcccatgtgctgggctgcttctcccctgctgagcaggagctgctgcctctgttgctggatcgagccaccgacctgatcttggaccacatccgtgagcgaagccaggggccctcactggggccgtgacactagtggccatggctgcctgcctgactgtagtgcccaccaacccagccactgccacagagctgccacgccagccttggtatctactttttatacaaatctcctctagactgttccaggctgcctgcggattaaagtgggggtgactgtgactggaccagtccatttctggagtaggttcttctctctgtgtcctacttgggacgtaggggaacttcaggaagactaaacttttcaagcctttttagagaaccaggggcacgcatctcagggctgctgtgtgcccggaaggtccccacacgggtgatatatgacagcagcctgaggtcctgggggttgggtgggatgtggacctggcgaggtaccaggcctagatcccccggctggtagggggtgatgtcagagagctgcggcagcagagacccagtcctgggcagctggatgctgggccggctctccttgggtgggccatgggactgtgactcctggtggggacacgcagccttctgaggtctcgtggccacagtggagctgagcatgaccagcagttgctgcagcatctccttgtgccatggctggaacgtcacgtcaacgtcactgtcctcttcatcgcggtgcatctgcagaatgttctgtaggaaggaggtggcctggaccagagccgcctccaggctggcccgaaccttctgctcattagccagttcctgctgtagccgctgcaaatccacctgctgctgctccagctgcaggctcagctggtctctctggctcttcagtgcctggttatccacctgcagctgcagggatctctgctccaactggctcagcaggaggcgcagctcctcggcctccttggtgtcctgctgctgctcctggcacttcttagtcagcatgaggatgatcttctggtggcctcttttgtgcctggccatgaccttctgggtgttctccagcagctccagctgtttgcacagattgttctgtcttcccttgagctgctcattctcctgcagcagcttcatgccttgctgggagaccctggccatctgcagggtaatgccgttgttctctttgatggcccgcttggttgtctcccacatccggttcgtggtcaccttgtggaactcattggccacgaggttcacgcgctggatgatctctttcctcagtctgtccttgtccagcaccgacttcttctccaggttgtatgcatagtccctgaactcattctcctgcttccgcacctgctcctccagcaatgtgaacttgtccgtgacctcctctttctgcagccggaactcctccagggctgccagcttccccccaaggatgatgttctccgtggtgagctggtccttggtctcctggaactcgtggcgcacctgggccagctgcgcctcgaaggcatccttctccatctctttggctagctgcaagttctggagctgctcgttgaggtctgtgatctcatccacctgctggttgagcgtgcgcttgaggaaggccacaatctccttcttgttattggccagctgctcaaactcctggcggaacatcttctcctgcacagccagctcatcccacttccgctggtaccgggctagccggtcctccaggtctcggatctggatgtggtagaactccttcatctccttggccagaggcggctccacggccaccaccggctccttcttgccccctttcttcttgacttcaagctccttgcctgccttgctcacactctttttgggagccatggctgatggcaaccagggctccaggccccaggaagaggccaggt

SEQ ID NO: 18849 - RNA, 2162 nt, Homo sapiens
  source 1..2162: mol_type = other RNA
tgcaggggtcgggtgggccaggggtcccccagcacctcgccaaagcttcctgggcctctctggctctcccacaggcaatgccaaggctgcgggtgggtatcgggcgcccggcgcaccctgaggcggttcaggcccatgtgctgggctgcttctcccctgctgagcaggagctgctgcctctgttgctggatcgagccaccgacctgatcttggaccacatccgtgagcgaagccaggggccctcactggggccgtgacactagtggccatggctgcctgcctgactgtagtgcccaccaacccagccactgccacagagctgccacgccagccttggtatctactttttatacaaatctcctctagactgttccaggctgcctgcggattaaagtgggggtgactgtgactggaccagtccatttctggagtaggttcttctctctgtgtcctacttgggacgtaggggaacttcaggaagactaaacttttcaagcctttttagagaaccaggggcacgcatctcagggctgctgtgtgcccggaaggtccccacacgggtgatatatgacagcagcctgaggtcctgggggttgggtgggatgtggacctggcgaggtaccaggcctagatcccccggctggtagggggtgatgtcagagagctgcggcagcagagacccagtcctgggcagctggatgctgggccggctctccttgggtgggccatgggactgtgactcctggtggggacacgcagccttctgaggtctcgtggccacagtggagctgagcatgaccagcagttgctgcagcatctccttgtgccatggctggaacgtcacgtcaacgtcactgtcctcttcatcgcggtgcatctgttggtgagggtggggtggcagcaggcccacagtggccccagtacccaccctcgtccaggaaattccaacctcagtgcccatttccacgaagttttccctgtctgcagaatgttctgtaggaaggaggtggcctggaccagagccgcctccaggctggcccgaaccttctgctcattagccagttcctgctgtagccgctgcaaatccacctgctgctgctccagctgcaggctcagctggtctctctggctcttcagtgcctggttatccacctgcagctgcagggatctctgctccaactggctcagcaggaggcgcagctcctcggcctccttggtgtcctgctgctgctcctggcacttcttagtcagcatgaggatgatcttctggtggcctcttttgtgcctggccatgaccttctgggtgttctccagcagctccagctgtttgcacagattgttctgtcttcccttgagctgctcattctcctgcagcagcttcatgccttgctgggagaccctggccatctgcagggtaatgccgttgttctctttgatggcccgcttggttgtctcccacatccggttcgtggtcaccttgtggaactcattggccacgaggttcacgcgctggatgatctctttcctcagtctgtccttgtccagcaccgacttcttctccaggttgtatgcatagtccctgaactcattctcctgcttccgcacctgctcctccagcaatgtgaacttgtccgtgacctcctctttctgcagccggaactcctccagggctgccagcttccccccaaggatgatgttctccgtggtgagctggtccttggtctcctggaactcgtggcgcacctgggccagctgcgcctcgaaggcatccttctccatctctttggctagctgcaagttctggagctgctcgttgaggtctgtgatctcatccacctgctggttgagcgtgcgcttgaggaaggccacaatctccttcttgttattggccagctgctcaaactcctggcggaacatcttctcctgcacagccagctcatcccacttccgctggtaccgggctagccggtcctccaggtctcggatctggatgtggtagaactccttcatctccttggccagaggcggctccacggccaccaccggctccttcttgccccctttcttcttgacttcaagctccttgcctgccttgctcacactctttttgggagccatggctgatggcaaccagggctccaggccccaggaagaggccaggt

SEQ ID NO: 18850 - RNA, 2627 nt, Homo sapiens
  source 1..2627: mol_type = other RNA
tgcatgacccttccctccccacagggaccccccatgtcccacacccaccctggtcaaaaggggccccttcctatgtgacttgccctgttacccccacccctaccctttattccatcagatccacactgtgtgccctcaccagggtggatgggcacccccaggcgtgtgggctcatccccctgtccccccacaaaaacaatcttaatgtctctgtggaggggctagggagagagggcccagctccctccggcccatccctgggtcccactctgttgggtctaagatgcacagccactctctcccagccatgtgtgtgcccaggggatggggaaggtgccagtgcccctccctttggtagctttccccacctcctgttccctgtccccctgcccctggctcctggagagggaacagcctcgttccacgatctgggtgctggtctggagtggttctggaaggggatagaactggcctgaggctgagtcttgggggtgagccaggaggtctagccccacctggcacaggcagcccagggctgagggagggatgcggcaaggccggctcccgcttggctgggcaggaggtgggggcagaccaggggtgtcagcctcagccacatgcagctgtcagtgccccaacatcaagccggaagcccaggaaggggcgttttgcaactgcactgtttgagaaaggctctgaccctactcaccacagcttgcagcagcttctgcatttggccccaaggcagggggaaggatttctggttcccagttgcgggtggctgaggagtcccatactttcccaaggtccttctgggggaaaatcaagtccttgacccccggcccctctgaacctctttgagaaagtcccagggcccagaacctcttcaagaaagtcccagggcgcccacgtccttggctccacggtgtttggttggagttcttctaaagtttcttcccagcagaagactggcgagattgggagagcaggatttccaggattcctggaagagtaacgtgaatgctcctgggtgggcagacgcaggggtgggtatggatcactgtctgtcactgcccccatcgggcagtgcagagctgattcagacaccacggagatccctgtgctgatagtgctgaggcgctcaccaggtccctcaaacagccctgtgacacagagctcttcgtcacctttgtgcagacaaagggtgttaaataactcgccaagaccacacagctagaaaatgatagagccaggactgaaacccaggtctgtgactccaaatcccgggctcttccccttccgggtttcccatcacagacatctactttcatgttggaaaaccttctccaacacccgcttccgtgttcgtggcggattgtccattcatgtccccaaccccagcccccgtctctcctttcccccagagcctgccttctcctgggcttccacagcttccctgccactggccaccaaaacaaagatggagctgttctgggagaacccagacacttcaaatgagcgggacttgggaggctgcagtgtggttggaagtggcatgcagctgagggaacagtctggaagcttcatttgcgcagcaaactcacttttttttacataggctgtttctggtctagtttgatgagaggtactctgagggcgactgaggggagctggacccctccaagctaccccttggcacctgcacttcttgccagggttctaggagggctgatggggcaggcaggggccaggaagctggacctctagggaagcaagtgctgcctgccagggcccgggtgagggtggaaagctgcagattgtgtattcaaggaaacaacgcttcactgtgccaaccgagcccaaccccgccgccaacagacgggctctcgtggaagacaaacccccgttctgcttccgctgtccgagtggggctgcagcctcctgggtccaagcagggtcctaggatcaaagccagggcatcagagccagggctctggggagagcagagggcagagaggaggggagcctgccctcctgggaagccagtcactagagcaggaggcaggagaccatgaggtcagcaggagaatgggagccagcctttccttgggggccaggagcgaggaacctgggcttccatcctagtctgcttgtcctccctgggcctcagtctacccacctgtaaaaggggcaggctatccctcatgacccccaaaggtccttcagccctgacctgcgtatgtctgaggggtcctgagcccttctggatattggaactgccttccagggccttctggtccacccctccgtgttgattcagcaggtacttcctgaggctggagatcgagggggaagagaggggatgggggaagatagacagactgtcagccatcactggtctcacacctagagtcattcaggttcctcctgagagagacctgaagggttgactccaacccctctccccatttgacagaagagggaaccaagacccagaaagatgtggcggtgacttgctcggggttacggagaggttctcagtgaggctgaaaccttgtatgatgaggagagtggtcccggtgtctcagggtggggctccgaggacatgacacacttagagttctggg

SEQ ID NO: 18851 - RNA, 1520 nt, Homo sapiens
  source 1..1520: mol_type = other RNA
tgcatgacccttccctccccacccgttcagtgaaaggagactgccagcagggcaagggtgactcaagtccaactaggcccaaacctctggggtgccctcctcacccagctgcctggctaaggtgtggacgaagctcatccactgacccagaacttgcccacccctcagtcccagagtcagcaacagactaacccctgccctctgcccagcccggcgacctcagagccagggtctacactgagagctgggaaaggaagggggagggtgaaagaaagcaggcggaggcgcaggttcctggaaggcgtctttaatcaggatttggtagtacacaagctctccggattgtctgcattaacatacagggacttaaaaaggcacaaaatccctcgcacagcgacgcgtgacggcggggcgccccctccccgcccgtgcgcggccgtgtgcgcgtgggtgcgtgtccgtgtcccacccccgtggcggcgccgcgcgtgtgcgtgtcggtttcaagtgttggatttgtacagtactcgcagtctaggggcagggggctcagtgcatgcttttctacccgggcctggggccaccccccgacgccgctatgtacactaaggaggacgcaccccggagagagagaggaagaaaaaaagcgtcccatcttcgtgtgcgtgtgtgtgcgtgtgagcgtgtgtgtggttttgagtttttcgtgcatgcttccgctggccagggtcgggaaatagtgcaagcgtataatacagtattattgcagtacaaaatggggggtcgagggaaggacttacgatgggaggggaaggctcaggaataaaccgactgggactcaggacctccgcgagggtcctctcgctaatccccttcctatccctcccctactccgcccccaccccgcaattagaaggcgtctccttacgcaggaaggggctcagctgggccccggtgctgagtttctctctcctaccagtcccgcttctccgggggcaggggccagcccctctcctcgctcgacactgagaactctgagggcccggagccccgccccctcccccacggaagcccctccgagcggggagcggggtcgacggagcaagtgcaaaggaagcagatgttggtccctgagttttattttcgggggtgggggtgtgggaagagctggaaatgggggggcatgtttggtgacccccagggccctcagtggtggggtggggcaggggacgcggattggggcgtgggcaaaaagggggctgttgggttgctctgagagacctgggctcaaagctctgctccccctcaactctgggctctttggcatccaattgcaaggccaattattggggcggggtggggggcagcccgacgggcagtgaggtaacgggagtcaggggtggggcgacagggccctccgagcctggaggcttagccgaacgcctccgcctgtccccatccgcaccccagcctggcagcactgaggggagccccactccagcccgcccccgccccggggc

SEQ ID NO: 18852 - RNA, 1506 nt, Homo sapiens
  source 1..1506: mol_type = other RNA
tgcatgacccttccctccccacctacaagtgtgcccagcccaggagtggccctgacaaggctagggctgggtggctggattctgaggctgctagtagtccccttggactgctgttgtcaccacaccttatctcaacaaatagacagtggacgaatttgattttaagtgcatccctccaaatgtcctttgggcattgggcacatggatgggttcaggaaggggaggaaggagacttttcaccatgaggaagtgccaagatattaggggtacttgaaaagcagaccgagatagactgcaaagggctgacactggggcaggaggaaggatgtcttacccccctttggaatcactgtatgtggtggagaccaaatcagaaaccatcttggcactacccatacttagcttgaaccacagacgaatgcattcttctggctctcggggtttctagtattcagacatcttccagagtccttcctcatggccttcatgtgactgagttctggctaatggaacagggcagaagcagatcctttccagacctgaggcataggaaccttcaattttccatcctctttgcatcttcttttgcaatgaccttggaaccatgagtgagaacatgcggtgtttggttttctgttcctgtgtcagtttgccgagaatgatggcttccagcttcatccatgtccctccttgtcgatagttttgtagccacacatggtgttgacaacttctgtcgtgttcctgatgcagcaggtgtagggcaccccacaggccaggggtccaggggcactgcagtcgtggtactgattcttgctccaatctcggtagtcctccccgccacagcacttgaactgagggaagcaagcaggaaagaggagctgccgtcatcgcccaggccctgctcagacgacaggaaggggccctttttctgaacaaagtccatgatgtttttgaagtccagatcatcatagtagttctcaattcctcttcgaatgttgtcgttcaggaagtcaatggtctggttccggaaggtcaaggccaccacgccaccaatgagctccatgatgaggcagatcccaaggatgtacatgaatgcttggagaaggtacaggttgtcacggagggacgccagcacaccaatgaaggagaccatgaacatgacgacgcccaggaggatgaggatgatggctggagccaggaaggcactttcaagggttttatatttctgccgctcaacctctgcatagatgcccacagacaggaccagggccccaatcagccagaacacggtggaatagatgataagtgaaaacttgagccagaggtaggagaagcgcgcgcagtagcgcacctgctccgagtccccgcgcggcatcctgggcgctccccgcgcgggttacgggggctccggggctctccggctcggtccctcagccagcgctcgtggccccacctgcggctgccgggctaccagccccgccaccggcgttctctccgggactgaca

SEQ ID NO: 18853 - RNA, 1452 nt, Homo sapiens
  source 1..1452: mol_type = other RNA
tgcatgacccttccctccccacctacaagtgtgcccagcccaggagtggccctgacaaggctagggctgggtggctggattctgaggctgctagtagtccccttggactgctgttgtcaccacaccttatctcaacaaatagacagtggacgaatttgattttaagtgcatccctccaaatgtcctttgggcattgggcacatggatgggttcaggaaggggaggaaggagacttttcaccatgaggaagtgccaagatattaggggtacttgaaaagcagaccgagatagactgcaaagggctgacactggggcaggaggaaggatgtcttacccccctttggaatcactgtatgtggtggagaccaaatcagaaaccatcttggcactacccatacttagcttgaaccacagacgaatgcattcttctggctctcggggtttctagtattcagacatcttccagagtccttcctcatggccttctgaggcataggaaccttcaattttccatcctctttgcatcttcttttgcaatgaccttggaaccatgagtgagaacatgcggtgtttggttttctgttcctgtgtcagtttgccgagaatgatggcttccagcttcatccatgtccctccttgtcgatagttttgtagccacacatggtgttgacaacttctgtcgtgttcctgatgcagcaggtgtagggcaccccacaggccaggggtccaggggcactgcagtcgtggtactgattcttgctccaatctcggtagtcctccccgccacagcacttgaactgagggaagcaagcaggaaagaggagctgccgtcatcgcccaggccctgctcagacgacaggaaggggccctttttctgaacaaagtccatgatgtttttgaagtccagatcatcatagtagttctcaattcctcttcgaatgttgtcgttcaggaagtcaatggtctggttccggaaggtcaaggccaccacgccaccaatgagctccatgatgaggcagatcccaaggatgtacatgaatgcttggagaaggtacaggttgtcacggagggacgccagcacaccaatgaaggagaccatgaacatgacgacgcccaggaggatgaggatgatggctggagccaggaaggcactttcaagggttttatatttctgccgctcaacctctgcatagatgcccacagacaggaccagggccccaatcagccagaacacggtggaatagatgataagtgaaaacttgagccagaggtaggagaagcgcgcgcagtagcgcacctgctccgagtccccgcgcggcatcctgggcgctccccgcgcgggttacgggggctccggggctctccggctcggtccctcagccagcgctcgtggccccacctgcggctgccgggctaccagccccgccaccggcgttctctccgggactgaca

SEQ ID NO: 18854 - RNA, 2298 nt, Homo sapiens
  source 1..2298: mol_type = other RNA
tgcatgacccttccctccccacgtgacactcattccttccaatgcaaactctggtgtatccacactcacttctgcgtcaccggtttcccccaacaaggcacaaagggcgggtgcttccaaaggatcccttgctcctggcagcgggactttcagtgctgggtgtcttgtgcaaatggtggctgaaagcaggactgttagttcactcagacactgggatcttccttactcctgaagaggggcttggctccaggcccacagtactcgttgtagatgagcttgaagaggaagaggtggaagagggtgattagggaggccacgctgaaccagaagaggaagggcagcccggggtcctgctgggccatgtgctcatcatgggccaggatggccttgaggtgcagcgtgtgccgcaggtcctgcaggtgtgtgaggtcggtggagatgtagagcagtggcgtgatgggctgtgtcaccatgaccgagaaggtgtggcccgtgggcgccgaggtcagctccactggctcgtccaggcagcctgccttgcaggcatagatcttgacaggctggccacgggactccacggacacgtgtaggtagggcttgccctcggcatccgccagcacggccaggttgatatggtcgttcttgtagcggatgccatgcaatgcatagctgttgtgcagcacgtcggggtcggcctggaactggaggtggttctctgtgaactgcagccccccaaagctgagcaccatcccctgcaggatgcctggggcacccaccttcaccagccccttgcagccacgcttctggagggtcagcctccacaggtcagagagctgcaggatctgctggacggaggacagccgccccggccacaggttctcggcgtgcatggtggcgtgcccgctgaagcagtgatcttcatagttgagcgtcgactccatctggtctcgctccctgtggctcagggaggggctgagcagtggggctggcgagcaggagagcatgtaatagagcgtcaggttcacggtgaggccagacggcgtgtgggtgtcagtgatcttcttcatttccactcctgggctgaagagctgagcccagaggagctggtggtcttgaagcagctccgccgctggcatgtccaagagctccagcatttccttccgtgccaagtcctgcagcgccttgagctccttggctgctttgcttttgagcacctgggggttaatggggccagagacgtgcaccacccacagcaccgtctcatccagctgcgtcttgggagccacttggaggcggttcaccagcttcttggcggccaccaccaccaggtgcaccaacccagtgggcgtaggcggggaccggcctgagtagaggaggaactgatggtctccgaccttctccagggtactggtgaaggccttgggggctgggccggcagtgggccccacagtctgcagcgcggccacgcgctccgtggggttgttgagctggatgcgctgcaggtagacgtggggtcggcccctgtgcgccagaaagtcctcttgcagcagcacgcagtcgcggccggaccccgcggcaaggccagagacggaggcgggcccggggccggcggccacggggccaggacctggggaccccagctgcaggcaacgcacgcggcgcagaagcccctcccgcagcagcagcaccgcctctccagcttcagccagcgcgctcagcgggcgcagctgcacgaagggcacaaagtccggcgccacggcgggctcccgctccccgggagtcacccacagccgattggcagccacgtccagggccaggaagccgttggccaccagggccggcactccaggacccagcggtaccacctcaccgcgctcccgcaggccgcgccaggcgcgggtggccgcctccaggcaggcagacggctcggcggcgcccggctcaccgcgggaccagggcagcaggtgcaggccgcccgccgcccgccgcgcgccggaccccccaaaccacagaagcagcagcaggaggccaagcaggcagaggaggcggcgggcccagctgctcgacagcagtcccggcagccccttgagccgctgctgcagccacatcgggccgccaggcgcgggcaagggtgcgagggcggccgccgggcccgccgcccagcccaccggcccggccgcccgcgcctcactgcccggcccggaccgcggcgcccaccccggcccccgccgcaaccgccgcagcagccgccacccctgcttcctccttcttctcggtggcctccagccgtcaaacgac

SEQ ID NO: 18855 - RNA, 427 nt, Homo sapiens
  source 1..427: mol_type = other RNA
tgcatgacccttccctccccactaccaccctccaaacttgccttttgccagggctagcggcaggaactagccaaaaagcccctcaaagattactcgtttcaaacatagcagctgctcttatccgcttaccccttcgttatcctcctgctgctgactagaaattatgacaaaaatattgaaccaaccacgagccaggccctgtgcccaaaacgttacatctgtcccttacctgctttaacactcctggcaccaccctactcactttacagatgacagcgtgaagtctcagcgaagttaaataattggctccaatgcacccagccacaaagagctcaagtcacagccgcgacctaggtgtgcctgattccaaagggtttttgttttttgttttgttttgtttttgagatggagtctggctctgtcaccc

SEQ ID NO: 18856 - RNA, 428 nt, Homo sapiens
  source 1..428: mol_type = other RNA
tgcatgacccttccctccccactaccaccctccaaacttgccttttgccagggctagcggcaggaactagccaaaaagcccctcaaagattactcgtttcaaacatagcagctgctcttatccgcttaccccttcgttatcctcctgctgctgactagaaattatgacaaaaatattgaaccaaccacgagccaggccctgtgcccaaaacgttacatctgtcccttacctgctttaacactcctggcaccaccctactcactttacagatgacagcgtgaagtctcagcgaagttaaataattggctccaatgcacccagccacaaagagctcaagtcacagccgcgacctaggtgtgcctgattccaaagggtttttgttttttgttttgttttgtttttgagatggagtctggctctgtcaccca

SEQ ID NO: 18857 - RNA, 429 nt, Homo sapiens
  source 1..429: mol_type = other RNA
tgcatgacccttccctccccactaccaccctccaaacttgccttttgccagggctagcggcaggaactagccaaaaagcccctcaaagattactcgtttcaaacatagcagctgctcttatccgcttaccccttcgttatcctcctgctgctgactagaaattatgacaaaaatattgaaccaaccacgagccaggccctgtgcccaaaacgttacatctgtcccttacctgctttaacactcctggcaccaccctactcactttacagatgacagcgtgaagtctcagcgaagttaaataattggctccaatgcacccagccacaaagagctcaagtcacagccgcgacctaggtgtgcctgattccaaagggtttttgttttttgttttgttttgtttttgagatggagtctggctctgtcacccag

SEQ ID NO: 18858 - RNA, 430 nt, Homo sapiens
  source 1..430: mol_type = other RNA
tgcatgacccttccctccccactaccaccctccaaacttgccttttgccagggctagcggcaggaactagccaaaaagcccctcaaagattactcgtttcaaacatagcagctgctcttatccgcttaccccttcgttatcctcctgctgctgactagaaattatgacaaaaatattgaaccaaccacgagccaggccctgtgcccaaaacgttacatctgtcccttacctgctttaacactcctggcaccaccctactcactttacagatgacagcgtgaagtctcagcgaagttaaataattggctccaatgcacccagccacaaagagctcaagtcacagccgcgacctaggtgtgcctgattccaaagggtttttgttttttgttttgttttgtttttgagatggagtctggctctgtcacccagt

SEQ ID NO: 18859 - RNA, 433 nt, Homo sapiens
  source 1..433: mol_type = other RNA
tgcatgacccttccctccccactaccaccctccaaacttgccttttgccagggctagcggcaggaactagccaaaaagcccctcaaagattactcgtttcaaacatagcagctgctcttatccgcttaccccttcgttatcctcctgctgctgactagaaattatgacaaaaatattgaaccaaccacgagccaggccctgtgcccaaaacgttacatctgtcccttacctgctttaacactcctggcaccaccctactcactttacagatgacagcgtgaagtctcagcgaagttaaataattggctccaatgcacccagccacaaagagctcaagtcacagccgcgacctaggtgtgcctgattccaaagggtttttgttttttgttttgttttgtttttgagatggagtctggctctgtcacccagtctg

SEQ ID NO: 18860 - RNA, 706 nt, Homo sapiens
  source 1..706: mol_type = other RNA
tgcatgacccttccctccccactctcatacaactcttcctcatctttcaggacttggcttcaatgtcaccttaactggaagcttctctcactctccagaagagcttcccattgcacctgatgcatgggaaacataatttgatcatttttaagttacagtccaaatctttttgtacctgaataacatgttgcccagtcagtctctcttcctggattcacaagtctttcatggtagatccagctccagctctgtggccctgtggttggagaccgctgctcaagtgcatttgaaaggaaccaacccacgccattcttcagagtcatctttactgctgcagtggtcaacttgtagcacccctaagctcgcaggacatatgcttcaactggcatttcacaatcaacagtatgtggcagcttgagtcattgtgagctcacatcctggaaatcaccagcatcccatatcccattgcaaggagctcagcactgctccttggataaccaaacctattcccaaatcccatctgtgtgcgtctatctcctggtacccttcctagcatcaattctgtatttgtaggagtccaatcaggagacacaaaccactcaaaagtttaaactagaatgagcaagatggctcacacctgtaatcccagaactctgggaggccaaggtgggtggactgctttgagctcaggagtttgagaacagtc

SEQ ID NO: 18861 - RNA, 703 nt, Homo sapiens
  source 1..703: mol_type = other RNA
tgcatgacccttccctccccactctcatacaactcttcctcatctttcaggacttggcttcaatgtcaccttaactggaagcttctctcactctccagaagagcttcccattgcacctgatgcatgggaaacataatttgatcatttttaagttacagtccaaatctttttgtacctgaataacatgttgcccagtcagtctctcttcctggattcacaagtctttcatggtagatccagctccagctctgtggccctgtggttggagaccgctgctcaagtgcatttgaaaggaaccatcccacgccattcttcagagtcatctttactgctgcagtggtcaacttgtagcacccctaagcttgcaggacatatgcttcaactggcatttcacaatcaacagtatgtggcagcttgagtcattgtgagcgcacttcctggaaatcaccagcatcccatatcccattgcaaggagctcagcactgctccttggataaccaaacctattcccaaatcccatctgtgtgcgtctatctcctggtacccttcctagcatcaattctgtatttgtaggagtccaatcaggagacacaaaccactcaaaagtttaaactagaatgagcaagatggctcacacctgtaatcccagaactctgggaggccaaggtgggtggactgctttgagctcaggagtttgagaaca

SEQ ID NO: 18862 - RNA, 285 nt, Homo sapiens
  source 1..285: mol_type = other RNA
tgcatgacccttccctccccactctcatacaactcttcctcatctttcaggacttggcttcaatgtcaccttaactggaagcttctctcactctccagaagagcttcccattgcacctgatgcatgggaaacataatttgatcatttttaagttacagtccaaatctttttgtacctgaataacatgttgcccagtcagtctctcttcctggattcacaagtctttcatggtagatccagctgtaatcccagctactcgggaggctgaggcaggagaattgcttg

SEQ ID NO: 18863 - RNA, 283 nt, Homo sapiens
  source 1..283: mol_type = other RNA
tgcatgacccttccctccccactctcatacaactcttcctcatctttcaggacttggcttcaatgtcaccttaactggaagcttctctcactctccagaagagcttcccattgcacctgatgcatgggaaacataatttgatcatttttaagttacagtccaaatctttttgtacctgaataacatgttgcccagtcagtctctcttcctggattcacaagtctttcatggtagatccagctgtagtcccagctactgggaaggctgacatggtaggattgct

SEQ ID NO: 18864 - RNA, 763 nt, Homo sapiens
  source 1..763: mol_type = other RNA
tgcatgacccttccctccccactctcatacaactcttcctcatctttcaggacttggcttcaatgtcaccttaactggaagcttctctcactctccagaagagcttcccattgcacctgatgcatgggaaacataatttgatcatttttaagttacagtccaaatctttttgtacctgaataacatgttgcccagtcagtctctcttcctggattcacaagtctttcatggtagatccagtataacgtagactcagtgggatctctgagcttgttttcctgcaactagactgtccatctccagctctgtggccctgtggttggagaccgctgctcaagtgcatttgaaaggaaccaacccacgccattcttcagagtcatctttactgctgcagtggtcaacttgtagcacccctaagctcgcaggacatatgcttcaactggcatttcacaatcaacagtatgtggcagcttgagtcattgtgagctcacatcctggaaatcaccagcatcccatatcccattgcaaggagctcagcactgctccttggataaccaaacctattcccaaatcccatctgtgtgcgtctatctcctggtacccttcctagcatcaattctgtatttgtaggagtccaatcaggagacacaaaccactcaaaagtttaaactagaatgagcaagatggctcacacctgtaatcccagaactctgggaggccaaggtgggtggactgctttgagctcaggagtttgagaacagtc

SEQ ID NO: 18865 - RNA, 760 nt, Homo sapiens
  source 1..760: mol_type = other RNA
tgcatgacccttccctccccactctcatacaactcttcctcatctttcaggacttggcttcaatgtcaccttaactggaagcttctctcactctccagaagagcttcccattgcacctgatgcatgggaaacataatttgatcatttttaagttacagtccaaatctttttgtacctgaataacatgttgcccagtcagtctctcttcctggattcacaagtctttcatggtagatccagtataatgtagactcagtgggatctctgagcttgttttcctgcaactagactgtccacctccagctctgtggccctgtggttggagaccgctgctcaagtgcatttgaaaggaaccatcccacgccattcttcagagtcatctttactgctgcagtggtcaacttgtagcacccctaagcttgcaggacatatgcttcaactggcatttcacaatcaacagtatgtggcagcttgagtcattgtgagcgcacttcctggaaatcaccagcatcccatatcccattgcaaggagctcagcactgctccttggataaccaaacctattcccaaatcccatctgtgtgcgtctatctcctggtacccttcctagcatcaattctgtatttgtaggagtccaatcaggagacacaaaccactcaaaagtttaaactagaatgagcaagatggctcacacctgtaatcccagaactctgggaggccaaggtgggtggactgctttgagctcaggagtttgagaaca

SEQ ID NO: 18866 - RNA, 142 nt, Homo sapiens
  source 1..142: mol_type = other RNA
tgccaaccgtcagagcccagaaccctcgcccggctcccccggcgggctctggaggcgcgccaggcctcctggctccccgcctgaatgtcagcgcagggacccgcagggaagaccaagcccaagctccagggggtggaatgct

SEQ ID NO: 18867 - RNA, 415 nt, Homo sapiens
  source 1..415: mol_type = other RNA
tgccctaaatgccccttctggctatttcccttctcggtcacaaagctgaagagcaggctctgagggccattgcccaggggaagtgcagattcacaaacaccagctgtgtatggctaccttggatgttacctacctactgctggagtccacctgccttcccacaggttggtggttgctctgtgagaggcaggtcattctagatacctctccctgtgatcctgagccacacaggacaaagtcttcacactcagcacagacatctgggttgattcagtctagggcagccaggctgttctagacacagctggttctggaactgggctcagcatgtccacctcggagatgctgtccaggctctccacctgtacgtccacgcccaccgggatggcagggcctgttgggtgtctgagctctc

SEQ ID NO: 18868 - RNA, 1569 nt, Homo sapiens
  source 1..1569: mol_type = other RNA
tgccctaaatgccccttctggctatttcccttctcggtcacaaagctgaagagcaggctctgagggccattgcccaggggaagtgcagattcacaaacaccagctgtgtatggctaccttggatgttacctacctactgctggagtccacctgccttcccacaggttggtggttgctctgtgagaggcaggtcattctagatacctctccctgtgatcctgagccacacaggacaaagtcttcacactcagcacagacatctgggttgattcagtctagggcagccaggctgttctagacacagctggttctggaactgggctcagctgttggatatccaaaggggctggcaatgtaaaatctagcatcttggaaactgtcatacctgcacctttcacacctgggccccatattttaccaggtgctggagctatggggggtgtacaacctcagtatcaatcatatcagctctgccatgctgggtccgttaggagcaaggggcgttcccactcttcaagggcagatgacagcattgcaagtgggatgcagtgctggcaagtggagcctccccgacttttatttattccacacattttcagggcccctgggggaccacactggactagacttggagatattggggtaaagaaaaacatgagtccctgcattcatggagcttatagtcaagcatggaagacaaccaatatataagaaaactccccaaataaatatctagcacaattataaatgatgatgtaggctatgaagaaaaaacagaaattctttagatcaggaggtcagggaagcctctttgaagaagtctcattttagctaagtcctgaaggataagaaggagatagctatggggagggccagagctgaagcatgctcaagatccctgaggcagaagaaagaggaagtttgcaaactgaaagagaggcatacagaagaaggaagagaggaggctggggccctggggtggggggcacacctctccactgtgagccttgcaggacacccaggcctgtggtggtagaattggggtagacatggagtgggggacactgccacaaagtgagtagggggactgcacttgcagcaggaactgaacatcagaaagctgcaaaatttcagcctgaaactgtccacctccagtaccccaccaggtgtggttcgcctgatcacttgcattatttgtggagtgtgttgaaaatgcaaagtatcactcccagagattctgaatcaggaagtgtgaaatggggcccagaaacccacatttaaccaactccttaggttatttttacccacgcagcgagaatgcccgctttagattttactgctccagggccgacttccaagcgcccattttatcacctccagctcccgctctgcccacacaggcacagcctgcaccaccgaggcccactacactacaggctctcacgctgtgtcactggaggccgctgcataccatgtccacctcggagatgctgtccaggctctccacctgtacgtccacgcccaccgggatggcagggcctgttgggtgtctgagctctctccacaacg

SEQ ID NO: 18869 - RNA, 451 nt, Homo sapiens
  source 1..451: mol_type = other RNA
tgccctaaatgccccttctggctatttcccttctcggtcacaaagctgaagagcaggctctgagggccattgcccaggggaagtgcagattcacaaacaccagctgtgtatggctaccttggatgttacctacctactgctggagtccacctgccttcccacaggttggtggttgctctgtgagaggcaggtcattctagatacctctccctgtgatcctgagccacacaggacaaagtcttcacactcagcacagacatctgggttgattcagtctagggcagccaggctgttctagacacagctggttctggaactgggctcaggctgtgtcactggaggccgctgcataccatgtccacctcggagatgctgtccaggctctccacctgtacgtccacgcccaccgggatggcagggcctgttgggtgtctgagctctctccacaacg

SEQ ID NO: 18870 - RNA, 15616 nt, Homo sapiens
  source 1..15616: mol_type = other RNA
tgccctcctttcttccctcattatagtcacctttcaataccatcaagcagtcaacagtatagaacaaaggatgcaagttctgcaggccagcatgtgaaatttaaaggtatttttaaatagcaagaataaacacatctgaggccagggtctaaagtgagaaaagacccaggactgacttggattctgagaacaaaactggatggaagaaaagatactggaacttgttttcactcactttggtggaaggatagctcctcttgtaataattcactgaccaaggaaggatctacagtatctgtgttaataaagtattgtctgggtggaaaaatttgaatagaaagaatgaaaaaaaatggaccagctctttccctctggtccaggagaacacttttgagaaatgcaaagatgaagaagagaactaattgaaatgctggtcaatccctaattatcttttcctatgatgctctttggcatcctagacttggggagaaaagactgaactgctcttggattgagaaaggttaggtgatcgaagatacgaattaaaagagaaaccaacaccaagattttgcctgtatcatctcagtccctgcatctaaactttagtggttatttatcaagttatcaatgtggagcttgtgtttttgtttcagaaatttcagtatgccaggtgttttacaacatttcacggtaagaagtttgctggcaccacttggacttgtgtaacacaaaactgtaaagaaaggaaataatattctaccttcaaggaagtatctgttaatggtatgactacctatccgattgctagtcttcggactcttttcttcccaggtggcaggttccttgtcataatctgaaaaaactttcctagagataaagctgactcttatgctaaaggccaaactggaccaaagcaaaggatatggggggataaaaacctcaaactctacaactttttgaataggattttcaagcagagataaagtaggcattgatgggccatgtttttggctggggcaatagctgtgattcagcctgtcgcccaagacagatcaacagcataggcaatgtgcactgcccctgccccctgagatgggagcaaagcacagggagatagtggggtctccttttccctcttgtatttttccagatcaaagaattgagaattgctaaaatataacctagcaaacaataggaaaccccattccatacctttctttgttttctaaataatcatctccaaaaggtatagatgggatagctaaacaggatgcagaggatggtgggagggggacttctgatgtggaagagccccactggatggaggggacctggatcctttgcaaccccaggatggaggaagaagcctttggtaatgtcccatgtaaagccaccagatgggctgcaatagccttgactggatagtgtgcaaggtggggaaaggtgagtgcctggtggcccacagaagattcaaggttactattttctttttcttgcctttcatgtatgaactggagtctgccttcatgctggcacatgctcaagaccaaaggattgcagggaagtgttggagtccagagagagtgaggttagagatttttggcccagttctctttaaagctgacagatacagagatttcttcctagtaccaaaacctaccttccagcccatgacctgccttttcccaggccaggcccatgtttccccaagagggcaggagagaaaaccaggccaagctgaggtaattttgtagttatgtgtctccaaggaaaaggacatccattggcacaaagcactgagtaaaaaccctttaataacaaaataacattcatgatgtagctacttcagttgtctggaaaactcagcttacacttgattcaacataccactttccacaatgttaaaagaaaaggacataaaatggcataacaaaatataccttgggtttcataagacaagtcttcttggcaaagtgtaaccagccagacccatgcattgcctgtgattaaaaaaagggctgggtacactcatgtctcaaatactcctctactttctttggatcaaaaatggatttgaactttgtagattctacaatatctgcattaagaggaacagtttgtgggtttgtgagtgtcaggaaaactttgctgaaacaaatatcaattttattgtggaacaacatataaagctttctggaagattaaacactattacaatcatcaattgtcttacaaaagccaatttgaaaaattcttgtatctgttcccatctttggcagattaataagagaaaaataaaaagactatatatcaaagtttacattaccacaacctaatttataaggccaaataaaaatatgttgctttttattattcacgagagcacgttcccaatataccctcattgacagataatatgaatgctacactgtcagtgatttccaatattttgcatagcagactgctgcttttcaaccaaggttccctaggctgcatactcctatgcaaaataaagtgtgcttggcagttgatttggctttatgtcaagcattttggtttgggaaatatgaaactggagaatgggtctttgaacccaagtataagaaagaacaagtttgcccaatcccctgcaactgaaaaatagttttgacatatagaggcctcagataattgaaggatttaaagaagatggttttcctaaagtgggtttcaaaacttcttcttatattaccttttagatggtagatggaacattgttgggcaggtaaaaattaagtgagagtcacctccaagtctagggagggacagccatgatagctgcacatgtgaagttttgggaaatggctgcgtatttttgcccaaatcactggaacagttggtgggaatgtctaggagagtggacaaaagagaagtgggcagagaagagttagtaatattgatgccatttgagtttctactgggagctgacctgatcacaaaatacgagaagaaaccacgcatagtcaaaaatagccattcccaagcagagatcaaagagggccacagctagatgaatttgcatctacatatacatggccagttaggtctaagttcatgagcataaagccaaaataactccttttggtggaaattaaatatgcaaaggtgagtttttcaatactcgctttcaaatccctctcacatacggtgatatatttgggttatgaggatcccaatttgtggaatgcaaattggctaactcaaaaattaggaataacgtttctcattataaagctggaacccaattcaatgtgactcattttcagatcccaacagatgtaaagggtattttcgaggtgacacatctcccaataaaaccaatattaccaccgtctgaggctgaactgtgtacattttcacagtttaatgtatacacaactgttccacaactgctaacaaacaataggcgcccatgcataaataaagtccattgaaccaaaggggaagatctagttcaaaatgaaaaatgttgctattaagaccacaatgcatcacactgctaaatttttagcctcatgcataaaattatagcactgattggcagttgctaatcataatactacactgttaacacggaacaattaattgttcagaccaagtggcacaaatgtagaaaataattattcttttcaacagagcaaatgaacacagattgtttcttcagcaaaatatgaaactgtaaactttgggctcattctgcaactttccccaatccagcataaataaaatccaaagggggaaaaaaacatacattttctttttaagcgcaccttttttcatctattacaaaagcacaacctaaaacgtataaagcttttttttcttttttctttttttaaatcacagttaccaaaagaaacagtgaataatttattacatacgctataataacattactctaaacactattgtctatgaggtatatctgagaaaattcggtaaggaattgcgcggtctgcattgccaacatgcccaggttcatagtaaagctttggaaccgtgaagaactagaaaaaagggaagaacgagggaggcagaggaggagacatagagaaagaacctttggtattagtacaaatcttgttctttgcagggttgcattgcaaagcaccacagtacaataagcccaccaactgactgtatggaggcccagttgaagctgaggtattcacaggaagaattaaaaaaagcacagagaggtccagactggctaaatcgttgctttggttcaagcaaggcactcgtcccgtggttatgtcacactttgcaagtgaagcatgaggctggggggattgctgaggagaggtctgccaagtggggatgttttctgtgttcaggctgccatcgctctttctagatcctctctcgtatgggtgtggcagtaggaaagatggggaaggtgatgttcacttatagggagctctgctgctcaatgaattaagtcatctttgctctgtctcccagggattctgagagttctaattccaataggaatttaggaagaaaaccaaagcaatgtactctttggaaggaaggccttacaggtttgccttgtatagggagaagatgggccttgagcttgtttggacaggagggaactttcacataggatggtgcttgaaaacttcagaaagagagtaacagtgtttcctacagtttgtcaatctgtcatttatattcctctactagctatgctttgttgatgcatggaactgatgagttgattggtcccttcctctctttgcttctttgtctaaatgctctctttaaaagctcaaaataactacattatgtgaaatgcaaaatactagcactcaaaaagagccatatggactagaggcagatctttgcatttgtctaaaacccatttggtcaaaagctgagacagattcattggctaacacacaaatcacgttgatgaatggctcttaatagtgatttaatcatttaatggaatctaaagaaacttgaagaagaccaattaatttcatgagtaagaaggaaagagagaagcaactttaagtagccatttcttaaactggcatattcctctgtaattttggggtcatttttcatttaccacaaataaccctttagtatcaaatgatgtaaggcttaaacttctctcataaatacagagttggcttagaaatgaaatgtaaacacctacaactaaaaaggaaaaggctgaagagcttaaatgtcacatgtgccaatggtggtcaagttccctttcttgataaatactgactttaaagtacccataataatcaaagccaacaggccaagaatgaactttctcctcctactgaattaaaaagttatctatacaatgctttgtaatggaaaggttcaaaagtgatcacatcattgggatcaacatgtttttcctagggcaaaaatcccgtatgagccctagtatttcaagacaggccaccttcacgaagcaaccgaccatatgtgactatgtactaatgggacactgaaaatgcttgtgactaattttacagctgaaaatgttaagagataaaccccagtccctgctcattgctaaaggattgccaccatcctatttgtcaatgtgggaccgctctcatgcagaggtagcactgtacaataagcggagcactggggcaggaaccaggaggcatgtgtgggctttcactctcaagagttatttgatttggataactatttcattcctctgggccaccggggcttggactaaatgattcctaaggtctcttccagctcaactactcaatggtcagagcttctgtggttcagtaattggcagtctttactgtgacaggtcccagcggggatagaggccatggctaggactgaaggccatttccaaccagtttccttcctcaatttgtaatcagaatttaaggaatccaattacagcagcatctgaactcgcatcttgaacatgtcgagcagacagcaaacatataagagaaacacagaaaatatccctttccaaattagcagccgccgtcgcatagataattatttctttggggtatctgagctgtggctgtacataccatatgtcagagaaaatcgttcaaattataaaagagcacaagcaaaatgcagaccgcacagagaaagaaatctttggtatctttggtgtcatcaacacgattaaaattacaaatggaaaaagtcagtgaggtagccttctttggttctcactagaaatagaaagtttttcattttttttttcttttttctgctttttgtttttttccttttttgttttgttgctttacatacacacagagttcattcttggaagcagctagtgtaagggtttctctctttttgtttacgatttttttaaaatttatttttccagtttctgtatagaagccccgaaatccaggctggtgaagcagggtctcagcttatgttttctgaatgcacaggttcaggctgaatagtcattgcttgtccacaaaatttgctctgttgttctgacagcaaacaaactgcagtgctctctgttgttttaaattaaaaatataaactatacagtgcacctttcacagatgctgaataagttaaataaataagttacaatatgaaggctccgagggccacaataattaagaggtgaagttcgcctggtaccaggtggggctgcgaacttaagttaaataatttaaaaattgttacttagactattttaaaagttaatttaagagggaagaatatcccaaattctctttttgtaacctgtatttcttccctgtctgtaacagaatttcactgctttataaagcaaactaaacttcaagagtattccaagtagaattttgcatctctgatgcaccattggtctaggttttgataaataagtacaaggagtagaatcaaactaaggaaggatgattaaataattacccaaatcctatacatttatgtactaggaactaatttaaataagttaattacattaatggtacttagcttgttgggtcataacccaaagagacaagataaaaagcattctgtggggtggggcagagggtgtcttcattttttgactgacaacatgtataacttcatttgatagtctaaataaaaacaaagcaggaaattataacctctaaaactttctcatgttaaagaccatttagatgtgacaagcatgaaaaaaatcaccactccccactagctaacgcagtctccccaagaccgcagtaccattgtctcaatcctggaaaccagagcccactgtctccccatcagtttgcgcttgactttattattttttcttctttttctttgttttttctttttttttttttctttttgtcctttttcaggtctttggatttagctttagttatgaaaaatccagaataaagctattcaaccgaagtcatcaatcataggtgtcatcctaacacagatgattaaataatatacaagatttcttgaaagttgagtttatcttggatatgcccaaatgaaattaattccaagtgtacaggatgaagatgctgggatacttttgttttccctgcactgtggttttcaatgttacaataaataatgaaaacaatgtacactgtagaagtaccacatacatgttaaacgatgatttaaaatttatttgttgtaacggattacagtatatacgtatgaagcttgtctgtacacacttgtatgtacacagtctagacacctataggtaatgtgtgttgttataaagtcatctatgagaacacatgttaaaatatgtatctaaatttgtatacatccaagcggacagactgtataaaccttaggcacacttatctgccaaggtttatgctacatgaaatgcttgctgctaaaaatggagcagagtggaagacttctatgggatgaacaagctggtagcaatgtctttttctccactagaaaaggtattagctggttacttccaatcaacctaactccaaaacctccaaggaaagcttgggctctagcaataactgcttcaggctgtcagagtcattttggtgtgtgagaataatgagcctcatttaaggtcctgtgtgattcacacaacagcccatcagcctcaatggtaagttctgtatctacctatgtgaggtcctatatattttaataactacttctgtattttataagtattctgagactttctaaaacagataaaccctcccctctttccctccccgaccttggaaacaaacaaatcattgatagaaaacaggcattgagacatccatatttaaaatcaacatcattatcttatgagacttatacaaccaactggggtgccattcttcattccgtaaggatttttgtggccttattttaaaactagaatctcctgttgtttcaggggtgacttgatcttagctaaagataaaaaaattactaatatatcaagtttggcagacaaatatcagaaagttatagatacaccagctctaccccttcttcatctaccatttccacttactcttcctggttaggctgagaagtctgaatcacacagcatcagcaacaacaaaaacaaaaagtcagctctaacctgttacgaatctagaagattatcgccaaggtagttgtgcctgggccttgtggtcaaccttgaccacatgtattatctttttctccactttttaatagagttcattattcttcaacaacattggaaacaggccttttcttcttagattttaaaatatccaactattcaaactcctgaaaatccgagttcactacaaaggcatactgtcatgacactttggtaatgataatcaaacagacattcctataattctaccaacattttcaaaagtggggaagtttcccccatacccagataatagtgattttaaaaatctgttcaacttgaatttactggcactagtaggtgggtgcccagtatagacaaagaaaataactgattatctaaaaggtatttatttttggttttgaaatatgttgtttgacttagaaaagtgtgtgtgtatcagatttacattccaaatgttgattttattttagcttgaattgaaaattattctggatttgctaaagcctacaattgccaagagcctgcagggggaaaagggagcttagaagcaactctttctggatttctccagaggaagtgccatgcttcctggttcaactagcctgcacctttatgcatggtgcaagctaaacacttcttttacattttggaaaagcttttaaatattggtgctgagtttttattgttgttgctgtttcctttaaaaaaagaaatgtattggctctgtctgtttttttttattatttcctggaatgaaataattatatccctagtaccaaaatcacattaaaacaaaaacaatgcaagcctatttgtgtaaaggaataaagtaaattgtttttccactcaatggctctgagtgttttgatttctgttgcctcaagaatgtgaaatttggctgagaactgttccttcacactgtaccttttcctgatggttgaggaatgcctggaattttccttggattgaggtaatggatactaaactataaccacacccaaatggttattttctctgaaattattaacttaaatttaaaaatccttgagtaaactcactgggttaaattctattacctttcaatatagaaatttttttctgttagatttctaacaaattgaaattctgcagggcttaaaattttgatacataactgtatagatacacatatatatttatatatgtatgtaaataattttctaaaagcaagcacttttctctggtatgacattatctggaatgagacatttattaaagctccttggagagaaattcttgccttttttttttttttaaacaattatgacatgttcttctgattatcagaggactggtttgaccaatgttgtaatgtcaggtcacaaaggcagcctctactagtctagacatcttcagaggatgctggagacccaaacgctgagattagtatgtcaaagaatcactaaccaaatcaaacaggctccattcctcaatccagtctggaaaagagcaaccatttccactggacacatgtcacaaggactcttttagaaatacccaagttgaaatcaacccacatgggaacactcctctgctgaaatatgctcttttcttagtcctttgacaaaggaaacatggagtatgagcaagggacaaagggacacaagggaagagccaatgaacaatctcctaggaaggatgaattataaaaattgtggagagtcacattctctcacagctcctgcatagggagacccacatagggggaatgaggagggggcacaaagaacaacaatggggctctctaggggcaggactccagaagtctccccaaaacctgctttatattttctcttcaggattgagacactctcccccatcccacccaacaccactgcccaccccagtgccagctgtggttgcacataggcttgtcaaaatacgaattggtaattaccaccctgaggaaatctatcaacccattgcaacaggagttgggcttcccctgtgagaagtccctttggtggacctgctcactgagggggtctggcacacccagatgggacagggcagctcctggagaacagatttctgggctggcctcatattctttaactggtgaaaatggaccaccgagccttcccaacagttacagaagatgagcaccccactgtcaggacccagttctgggccgagtctgttggatgcacttcactcaccaccttaatcgaggctgagggatagaatagagatgactccgaatacaaataaaactcatgtacaccatggatccatttatcaacaggttaaatgctaaaatgcttgatcttgactttaaacctgtcccagaaacttccatagagatctgaatacttcaaatcatccacagtggcaaattaactctggaatggcatgagaaatgagaaaaattctgaaccgaatacttagcaaatgaagcactggaccaaaacaagacatgaatttggacagcaataattttggttatcaccaatgtcaagttgatctatatatgtattttatatattatatatatctttctttagaaatgcaactttacagctgatttttaaaaagctaatagaaaagtagaaactggcaattatttttacatgtttccccccacccccaaatgaagccctgttaggatgtagcaatcacatgaaaacgaggctgtaaattcctctataaactctttggttctgtggctcgggagaggatgcatcaccaagacccctatccctgaccctcactccctttccttcccctgatgatgagactctgaacatagaaggaaccaagtctaagggttaagcaaagaacattcaagtgataatgttattccctaccctctgctgagcagagagaactgttcaatatcccaacatcttaaacttggagtccatggaaacttttgagagattccatgttggggcaaaaaaccataagacaaaattgaaatgaaacaataaaatcaaataaatggccctttccttttgttgctcagagaaacataattgattacctttatacagttcaatggcgctattagtattttagccaggcaagaggagataatgaactgaaacaaaaggtgtgagaaatcctcatctttggtattgtagctgttgaggtttctgttgctctgttccgtgttcttttgaaaaactgcataggcacaaattaaagacaatcttcagctttaagattaccgtgtgagttgtcaaatgaagcagcagccactgaggctcttccttatttctatctttgtctcaaccctttctttaaaatctgcttccaaaaaatgtcccaagaggtctgtttgaacacagtgtgtctccctgtttttgttttcgtttattttctggcgtgcttccttcttattggtggtgatttccattgatttacggatttatttattcattttaatgggacagttttgtttgttgcagaagtaggtgcagaaaaagtttctttggtttcgactaagtaattcataaaaaagtcagtctcaagtgtctgtaaagaatgattgcagcgtttggcttgctttgaacacccccacgtggccccacccggggccattcactggtaaatatgcacattgtgacctttgcaatctcccagagttctgtgggcgctcttccacttgctatgggaaggtgacaactggtgtggcaaagccacccctctgggtggcttggctaatgtccttggtgtagctggtccgctcagcccgatgatgcgccaaatgcaagagctgaatgccattcggagttgcagaggttttctgatttctaaaagtaatcacagtatttttaggctagaaaatgacaagtcataaatgtctttggtttgcagtattctgcttctttggtgtgctgtgttttctccagatgtattcagctgttttgcaaggatgattcaacaacagaagagatttaggactagatgacagtcatgagtaacatgtatgcaggtttgattgattgatttttttttcttgctagaaaacacagaaaacatccctactaatgggatggatgaggaaaaaccccaaatcagaaagagcgagaatggattacgtggtggtcataacacacagtaggagggaccagatgactgatcaaccaaggacacattaatgacctaaaaaaacctagatcttttaaaatgctgcattcgctccatgcactgttaacagttaaattggcctcctgagtgtgcgtctgcattatgtacaacagaatttgtagcaaactgcaaaatgtgcttgaagccatattctcatcaattccctaatgacttcacaataggtgtcttgaaaatccagatgtagtgaacccagaaccttcctcacttctgtttatctttgttgtgcttgatactttgagcgcaagtgaactgactggtttttttgacggatccaagaccatatgagatttccaggaggtaaagaaaaaaaaaattgtaagctggatcaacttaaagctttctaaatcattcaatgaaaagatgtctgggttggaaaaacaggtccttggatttttttttttaacgtccatatttaaaacttgtgctcagtaattaccattctgatgttgtggctgtgaacttggacataacatggtataatgaggctaagcatgtggaaagcaaatgaggtcattctcgttgctagattcttctcttattgttgtatcttggaagcctaaactcagagtccttacataggccaaactcctattgttactcataggaactctgactgcaagaagctgacaggacctgaagtgggatggatgatattttaagcaatcccgagcttggttgacaccatactggaattaactcgctccaggaaggccccatttgggtttctgggatgcttagcatgctcagagaacagtgtctggttctaagagattaatttttcagcttgcacttggactccatagccattaaaaacaaaagaagaacacctggcctatgattacagctagaatataagtttctttgcaagagaattgtgctttcaaatcaccagtgaagggccccagctaggaatccggtgtctttttcctttgttttcttttggtatctgttgtcctcatttggaggtgacttgtgcccaagtgagagtccttccatcatgctttggtacacgtgctggaggtggacgaggagccccctgtgctcagatcgtcttgccacttctccaggctgcggcgccgggcgttcatgaagaagttgctgacggttgtgagctccaggcccagctgctgggaaatggtgatctgcatctcctttgacgggcgtttgttctccttgaagatggcgaagagtgttcggcgttggaggtcagtgaacaccaggcgggacttcttctgggaattgttcctgtctttgtttggttcttgctctttgcgtttgcacgctgccaggcgtaaggcggacatgcgctggaactcgggctcctgaagccacttccacatcctgcggaaggtctccctgccagatttgagtttactccacggttttggattccggagcaggtcggagagagtcccctgagaccggcacagcaccctctgcgcaaagatcgcctgggggatactgtagcgcttcagctccgctgtgatgcgctgggccacctctttggtgttgatttcttccagctggcccgacgtggccacctgcgagcccgatgaggacgagggtggccgctcgcgactgggtgccagcaccggcccgtgagactgagtgtggcccgggtggtgcaggccgttcaggtgcgacatcatggccgcaggtggggtgcccaggccgcgggacaggtgttgctcaccgcgggtcagcatggcagtgtggtgcgcgtcgaagttggggctgagcattttgtcgtggcccggcggaccgtagttgggcagactctgctgcgcgttgtggaggccgcctagcccgttgcccagcggcgtggcggccagcggggacaggctctggctcatgccgggcatctccttgtagggactgtagaggttgttcatggccgggagcccgcgctcgtcgcgcatgagggtgaagctgccgctgacgttgccggacaggcgctggtggtggtggtggtggtggtggtgcggatggtggtgcgggtgagggtggtggaacttgtcagacacggtggagatgggtggcagcggctggagcggtgtcagcgtggtgtaggtgttgctcatgcccatgccaggcggagacgagtcgcaggacatgctcatggcgtggtgcagcgggatggagagctcgggccggtagtcgccgccgtccaggatcgaggccatgctggtgaccatggccgagcgcgacgccgccgctgccgccgctgccgccgtgcccagctcctggtgcgcggttggaggcggcggagggccccgcagcgagccagcggcgccgcggcccgcgtggtgggggctggggctggccagcagctcctgctcatggcccgggcccccgccgccgcccccgccgcccccgccgccgcccccgccactgccgccgccggccggcccgtgcaaagtgcccagactttccattgtcagctccgggttcatggcgcagccttctaggtctttggtgaggcatcgataggcggtgtaggcagccttcattcagtccatcagggcccgggggcggcgggggcggcgggggcggccggcgggcgggcaaggcgcgcgtggcggggctcggctgcgggagtgggggcgggcgcgggagtgagtggagaggagtgcgcgtgcgggtgtgcgccccgggctgcgggcgggctcgcccggggtgggggcggggtgggggcggacggggcgtgcgtgcgggagaggggaggggacggggagggagggagggatcaccgggccccgccgctcgggccggctcgcagcctcgccatgtccgagcccgctccggcgccgacgtcttctgtttgggtgagcgggagctgtccagaagggctct

SEQ ID NO: 18871 - RNA, 304 nt, Homo sapiens
  source 1..304: mol_type = other RNA
tgccctcctttcttccctcattctaagcagataacctggctcatctcattccctgaaacccttcctatagacccacttgcatctgcaaccatctcttccttccttcttttatccactggaaagttaatctcccccaagggccctggatcccacttcctcctctcttctcttgaccctagctccatcaactgctatctctctttcatgtacctgcaacgtttccctccctttttgctgcttttcctcagcaattttttttttttttttgagacagagtctcactctgtcgcccagctgggagtgc

SEQ ID NO: 18872 - RNA, 343 nt, Homo sapiens
  source 1..343: mol_type = other RNA
tgccctcctttcttccctcccagaatcatgtaaaatgctgacttctaggagaaagaaaaagcaagcctcatcttccatcctaaagcagctcctctacctgtttctggttgggagaaacaggatgtttcatcgcaggctgcaatcagtcctgttatttggcccagagtgagccagggcctccccgcagacaactgcccgctccagcattgcctctggatggcaagatgtaccccatcatccaagatgtctgcctgggctctgatctgctctgttcttgctttcctccagggacgggtggctcagtacctcacagaagcaagtcctgccttcttatgttggagat

SEQ ID NO: 18873 - RNA, 625 nt, Homo sapiens
  source 1..625: mol_type = other RNA
tgccctcctttcttccctccctcttgtcatccacaatgtggcgagcaaggggcatgtttcaatcctgtttgtgttacagctattttagctccaccataccggcaagtcccaagttcttgtcctgtgtccaggatgaatgaggtaaggcagacaaatggagggcgagtaagcagaagaagacctttactgagcgacagaacagctcagaggagacccagagtgaacagctggtttccataggcagggcgtcccagtgagtgttcagctctcagcagagacgaagcccacagtgggtagctcctctctgcagctggtagtcctgatgtctgcttagctctcaacagagaggagactctggagtgcgtaaggggcaggaggcagagggccctcccagctcccaagagcacagagacttccgggaccacagccatggctgggcagctgcagctgcacccagaagggagaggatctgctcctgctcgctctgatccccaagcacagggatgcctggctccagggctgcggctcggtggccacaacagcagccagggaacaggaggctcccgtcctgccaactcacaaggaggcagggttttcacctattcccagctcccaccagctctgt

SEQ ID NO: 18874 - RNA, 135 nt, Homo sapiens
  source 1..135: mol_type = other RNA
tgccctcctttcttccctccttcattcacttcataagccccaaggaaagcctgtggacagacagatgatgtgatatatttcttcctttccattcttgggcagcttcttctctctgcggctgaaagcaaatgcatt

SEQ ID NO: 18875 - RNA, 376 nt, Homo sapiens
  source 1..376: mol_type = other RNA
tgccctcctttcttccctcggaagtcagagcttggctacttgaagcactgcgcccgcctaaggagggttttccacgcttcattcccagagccagaaaggcccaggagccttcctgttctagtgtcccatcgaggtgcagaaactttggaggctgcaaatcttctaatcgcttgcctaacctgtgctcccctacctagggttgccacatagaatacctgatacccagttatatttgaatttcacataatgaatattttttactataacccttatagtataagggatataccttaaaactgagcatcctgtaacttcgtgacatctggcaaccctaaccctacctatccactcagggcaggagaggttggttttaact

SEQ ID NO: 18876 - RNA, 150 nt, Homo sapiens
  source 1..150: mol_type = other RNA
tgccctcctttcttccctctttcctttgacctcatccacaggctgttagatagattgaccatcacaacgtgaagtctcacaatagtgagaggtgacagcgtgctgacagtcctcagagcccttgctcgctctcagcgcctcctctgcctg

SEQ ID NO: 18877 - RNA, 360 nt, Homo sapiens
  source 1..360: mol_type = other RNA
tgccctgagacttttgctccttttattgttgttgcagtcaagaactcagcagagaagagaagagacactcagctagggaatagaggaaaatttagtggagggactatttacagagatgtgggcaccatgtaagacccaagaggggacgttgaggcaccagagactagaggagctgtctcctttgtgtctgaaaggacaggggagagtacgatattatcagaggctcatcagagctggaggcctggaggaagtgcccgtgggtaggtgtttctctaaccatggagaagcacagcttctgtccaagatcaggcaatgcaccagggaggaagtggggaatccatgcctgatatggtttggatc

SEQ ID NO: 18878 - RNA, 5615 nt, Homo sapiens
  source 1..5615: mol_type = other RNA
tgccctgcatggtgtccccacagaaagatctgtctgtgtcccagaacctgtaaagatgaccttatttgaaaaaagggtctttgcagatataatcaggtcaagacctggcagcgtgatcgtcctgggctgtcaggctggaccacagcgcctggtgtgaaggacaagcgccttcatgaagagaagagaaaacccagggagagccacatggagaggggccgaggccgtgggagggccaggcagggactggagggaggcagccacaagccaaggaacgcctgggccaccagaagctgccagagacaaggaagatccccctctagcgcctctggagggagtgcagccctgcccacagcttaatttggggcttctggtccccagagctgtaagggaatcagtatctgttgttgaggccacctggcttgttgcaagagccccaggacacgcgcccacttggccacgttgcccaggcggttgtggtcgagtgcccagggttccggccccagcgcctgcactcctgaccacacaggaggttgacgcctgccgggaagtctgctcacggcaccctctctctttccggattccagtgcttcctgcggtgctctgtgcaaaggagtgctgccggctcccatccccagcctctcagggctgggaggtgacatccagcagcaagcaggggccccgctgtctgcgacagcgtggctgagagttggtgccggccaggtgtgttggctcatgcctgtaatcccagcgctttgggaggctaaggtgggaggatggcttgaacccaggagttcaaggctacaatgagctatgcttgcaccactgcactccagcctgggcgaatgtgagaccgtttctataaaatacaatagagagacggcgagtcggtgccacacgattggcccttggtgtgttttccctgcccatcagagctaccccaaggaactgagtgagcaaatgtgtgcctgtctgctcacctgcttaagatgcaaagtgtcgaaagcagggccccacccagcatcttcccctcccgcaggtgcctggcacgctgggctcctgccgccacaaaccgacgtgacttggtgaacgtaagtgagcactggctgaccggatcatgtttaaaggaatcctttaggggaaccactctgcaaagaaagtaaccctcagtaactcgcttttagttatatgtggacttcaccttatccggcttccataaggtggatttgcagaaagccggggcggtggcgcggcgggaggcgtgggagctggtgggattctccgcaggtgctgctgggccgggcagtggctccggtggggggcgctgtgtctccaggccctgacctggctcccgctgggccggctgtggcagggaagagccatttttcatggcaggggggtggcttcacaccggcccaagtgccagtatgttccacagttctttttgctgacggaatcagccatcagctcagcccaggtgacttccaacctaatctaaacaaggtggggtcggtggactcagctctcacaaagaaagacacggtgacgtcgggcgtggccacgtgaggcaggggtggggagaggctgacagcctctgcctctccctccaccggcaccgcccgccccaagctcacgtggcccttgcggacgtcattccttcactgggtcgtgccaagcagcaggggtgcggctgtcccagtcctcacgccctgccctcctcgggcagcctgggtgtccgctcctgcactcagagcactccccgccaggcaccccccgccaggcaccccccatccacacccaaaggcaggcccaggcacatggcttgggtgacagagtctgtttggggcgatgcctgcaagccctgtgggaaatcggggtggagggagcgggcggggccgagcggccgcgggaacgagcagtgccctgcctccaagggagccccgggtcctctccccactggctggccctgtcgtggacatgagctctcaggtttctgacgggctgagcgtagtggctgagggctccctcaggcaggggcaggtgggcttgggccaaagagaaacctcttccccgataggggacacagcagacagccaccaggagccggagtggaggggccaggctgtgctcagcctcacgacacactggcgttcgctcaagctcatggctggcgtttaggagggcaccgcgagcacctactgagctgggatgaggtcggaggctgcccctgcccagtgagatgaatgccccggggccatgtgggctcttggccgggtggtgccaggatgtgcctggatttcagagtaggtggtcaggggtggccacctgctgggagtctggaccgtggagccggggcgactgggcttcagcttcagtggctgcacaacatccaaaagcagggggcccttgaggacccagccctgctctccgggcattgggcacttggccccagcgccccccctttctcggtgcgaggccgagcatctcccaagtctggtgcccacccggctgccttggcctctgcccactccaagccagctcttactccgccacaggcccggcccctctcacttccagcctgggccccactgtcacttcccatcatctccctcctgggtgacagccttgggaagggtctctggcctagactctgatcccaggacacggcccttcctgctccttggtggccttcctgggcttccaagtccgcgaccatacccatgacctgctgcccgctgctggtgggcctcagatttcccggaaagagggaagaggctcagaccagcccatagcagctttccaggtgaggccgtgatcatgagcagtccagggtccgctgcctggtgggggcgggaccgcaggctgggcagggacagcaggcaggggtccctccccccacacagccccccctcctgtgcggggctctggggtcctgccttacaggggtcctgtgtcacctcagtggggagcaggagatgggcccggggctcggggctgccatctccactgcatggtctggggctgagctgtcgtggagcaactcgggccacatgtttgtaatttggggacaattctgtcttcctgtaattttattgtatttagtaaatgcggtttaattttcttcctgtatagacttctcaaataactacaaatcaaaaaagagcttgcagtcccttcaggggcaaccgtggcctccaaggacccaacagcaggcccgtggcacacactcatgcccgctcccactcccagacacttcacgcctgcactcacgcctcacagccacacacacgggcacacccacagtgggcacgctcacaccccagtcacgcacacacacacatccacacacctccctctgctgcttcctccctcaagtgcccgcacccccatgcgtccccgtacagtcccagtcagggccgctcccccgcaccccccgtcatttcccacttccgttcccagcaccggcattcggcatttgccgcgggccgagggctggtgcgacagaagccctgccagcgccacgagccgacgcccctgtaaaagcggctgttccgcgcacacaggagccgcctctggcctgccagacacgtcctgcccggaggaccacagacccgaggccggctaggaccagaggaccgcggctcactggccatcagcaggctcacagggtcccctcgcagcacccagggggctggggcccggccgaccactgagagaactcgccgtgcatcccctgccggcctccctgctcaggggcagctgggacgtgggcagccgcctttcagactctagccagggtcccggatgtggggaaggccacccatcaggcgagtgtatgtgagacgtggggacaacgggggcaccccacggagacaccagcttgtcctgccgcgttctccatgtgctggagtgggggtggctgcaggcgcagctgcttcccctggctcatctggctttcaggtggtcacggctgtgcgggtctgttccccagctcccgggggtgcaaggcagtggcaacgcagcggccctggtggctttatgctcccggcacggctccgggggggctgccgtggtgacagtgcctggtggggcggcactctgtgcctgagtctcccaggaggcccgtctggagtctgcagcccatcctgggtcctgtgataccccttccctgtgttcaatcccttcctgctcagagtccttgggtccacttttccctgcttggacccatctgtcatgaacccttgagtgggtggtgctgctgagggctggtgcctggaggcaccgggccagctggagctgggagggtgggcagaggaaacgccacatgaagaagctgcagggttctccattctggccacacaaagtgcccgcagtggataatgcttccaggggagtgggggtgactggagggttggaggggtatctggacagctccctgggggcagttcccttgtgagcgtttgtgggggtgaaaatccctgtcacgtctccttccagaatgtccattctacttcaatgccaagtttaagtacatggtgcctaacccacgccctctgtgtgcaactgggtgaggtcatctacccgctcctccaggtcacaacaaatccatccctccccagcctgtttccaacttgactgaaacacccctaaatgctccacaaagttcctgggcagccctgggctccaagaggcttggccaggggtgagcttaaaggagagcacacatgtgcacacacacggacccacccacagagacacgtgcatacgcatggatccacacacacaaacacatgtacacacaaactcgcatacacaaacacaagcactcacaaaatcacacacatgcacacagtaactcatacacacgagtacatgcctgcattcacctgacaacacaaacacacatgcatacggcaaacccacatgcacacacctacgcatgcccacgtgcacaaagcaaatatctgcacataaccaaatccataggcgtgcacaagaaaacatatacacagatacacacacttgcgtgtagtgcacacaagcatacacaaacacgcacacacgcaagcacagatgcaggcacacacggagagattttggttctttgctcgtgaatcatttgttcactaattaaatcacccatcagcttctttgacaagggcgtcatgtgagcctcctgcatgccagggtgagttctgagtgttgaagctcccacaggaaatggcaccgtcccgggagcaacagtcttgaagactgtggatggcttccttgtcttgccctggccagaggcggggccctgggttagcacaaggctttctcagatgaagttccaaagtttccccataaaaggagtcactccaagctagcgtcgcccacgacatccttccaggcctggctcccctgggccacgcggagtggagggggcaggcgggtctgtgcagaggaaggggcaccctccccgtgcagggaaggtgctctgctcttcccacccccgaatccagcccccaccccactccaaggcacccagctctgccccgccgccctcctgttcatcctttcgcacttttgggggcttggtggctttagcatggcctgtcccctccagggacccacccacc

SEQ ID NO: 18879 - RNA, 1925 nt, Homo sapiens
  source 1..1925: mol_type = other RNA
tgccctgcctgttttctcctttttcatttctgcccctatcaaaacttcttttctgccaggtgcagtggaccaacatctgtagttccggctgctcaggaaggtgaagtgggaggatcacttgagcccaggaatttgagtccagcctgggcaacacagcaagacctcattgctttaaaaaaaaaaagtagggctcagtggctcatgcctgtaatcccagctacgtaagaggctcaggcaggaggattacttgagcccaggagttcagggctgcagtgagctgtgattgtgccactgcactccaccctaggtgacagaacaagaccccatctcttaaaaacaaaccaaccaaaaaacacaggtttcgtctcagagaagcggggtgggctctacttagtagtagagtctcttaaaacaatcaacagtagtgtaatttatcaataatcagatagcagacatccctctcagagatctatatattttcagccacaaagcttaaaatctcaaatgtcaacgagtaggatttcaggcaaaataaaagtagaaaataaaaatcagaatgtagatccatgttgggagaggaggttaactttccaggtaattcatactgagattgtttacacagctcctgcgggtccggctttctgtggctttctttagctaaggccagaaattcaaaaaaatcccaatggttatggagatccctcctcacccatccatccacccaatgagaaagaagaatttgtggagggcaggggatatcacaagagaaaatggcacaccagggtgtaatgtctcaaataaaaggcttactttacacttaatactagtatattactgttcataataatatatcgtaaaattatcatgttataaaaatatataataagatcttataagaaactctgaatggattgacgcttgataattctcttaagtagaacacaatgaaacagtagtggctggctaagttccatcaattttttttaattctttttgactttttctcgtggtcttctgttatcctttctgcaggtcgcttcttcaaccccttcattttcctggtttgtagtttgcttaggtcttgcttctgcatatgaatccttccataagttgtaccaaaagtatcatgggaaatatttttcttcttctttggcttgagagcttttggcattttcatagataatttataaaggtcatccgatgccaggtgtgtcctcctcagaaccagatccaatgagggtcccatctcttccaattcaatccgtggtgttctgcaaccagatttcttcaacagcaacttatagcttcgaaagtaaatcttcccattcagtgcagtgaagtgcagaacatactctaatccagccaggcggatatttgatactgtggggcctctgaagaaatcaataagaagactttttagtcttctataatcttctgttacatcgaaatcatcgccagcaaatatcagcatgggttttgttccctcaggacatttactgttcttaatgtcttttagagagacaaaattctcaatacctaattcaatcatatccagcacatggtagtcatacatacgacctattactagattatttggccgcttcttattatgggagccaaacatgaataaagaacaatctgacttctttgaaaagaattccagtgatgtctgatcctcaaaaggtcttgtaatatttttccacatctttaagtacttttgtcactgttgcatttgcatttccccctttaatcagcatggcatttttaatattttcattgagtttcggttctctcttctcaaggaatctcttggctcttttcgttttgggctttactactcgatccagagtgtccatcgctaccgctacctgcaactcttaaccagggggcatgcacgtgccctcggcgattacgtgcgccggaac

SEQ ID NO: 18880 - RNA, 1963 nt, Homo sapiens
  source 1..1963: mol_type = other RNA
tgccctgcctgttttctcctttttcatttctgcccctatcaaaacttcttttctgccaggtgcagtggaccaacatctgtagttccggctgctcaggaaggtgaagtgggaggatcacttgagcccaggaatttgagtccagcctgggcaacacagcaagacctcattgctttaaaaaaaaaaagtagggctcagtggctcatgcctgtaatcccagctacgtaagaggctcaggcaggaggattacttgagcccaggagttcagggctgcagtgagctgtgattgtgccactgcactccaccctaggtgacagaacaagaccccatctcttaaaaacaaaccaaccaaaaaacacaggtttcgtctcagagaagcggggtgggctctacttagtagtagagtctcttaaaacaatcaacagtagtgtaatttatcaataatcagatagcagacatccctctcagagatctatatattttcagccacaaagcttaaaatctcaaatgtcaacgagtaggatttcaggcaaaataaaagtagaaaataaaaatcagaatgtagatccatgttgggagaggaggttaactttccaggtaattcatactgagattgtttacacagctcctgcgggtccggctttctgtggctttctttagctaaggccagaaattcaaaaaaatcccaatggttatggagatccctcctcacccatccatccacccaatgagaaagaagaatttgtggagggcaggggatatcacaagagaaaatggcacaccagggtgtaatgtctcaaataaaaggcttactttacacttaatactagtatattactgttcataataatatatcgtaaaattatcatgttataaaaatatataataagatcttataagaaactctgaatggattgacgcttgataattctcttaagtagaacacaatgaaacagtagtggctggctaagttccatcaattttttttaattctttttgactttttctcgtggtcttctgttatcctttctgcaggtcgcttcttcaaccccttcattttcctggtttgtagtttgcttaggtcttgcttctgcatatgaatccttccataagttgtaccaaaagtatcatgggaaatatttttcttcttctttggcttgagagcttttggcattttcatagataatttataaaggtcatccgatgccaggtgtgtcctcctcagaaccagatccaatgagggtcccatctcttccaattcaatccgtggtgttctgcaaccagatttcttcaacagcaacttatagcttcgaaagtaaatcttcccattcagtgcagtgaagtgcagaacatactctaatccagccaggcggatatttgatactgtggggcctctgaagaaatcaataagaagactttttagtcttctataatcttctgttacatcgaaatcatcgccagcaaatatcagcatgggttttgttccctcaggacatttactgttcttaatgtcttttagagagacaaaattctcaatacctaattcaatcatatccagcacatggtagtcatacatacgacctattactagattatttggccgcttcttattatgggagccaaacatgaataaagaacaatctgacttctttgaaaagaattccagtgatgtctgatcctcaaaaggtcttgtaatatttttctttttatatagtacaccgtatggttttttcagtgcatacacatctttaagtacttttgtcactgttgcatttgcatttccccctttaatcagcatggcatttttaatattttcattgagtttcggttctctcttctcaaggaatctcttggctcttttcgttttgggctttactactcgatccagagtgtccatcgctaccgctacctgcaactcttaaccagggggcatgcacgtgccctcggcgattacgtgcgccggaac

SEQ ID NO: 18881 - RNA, 2420 nt, Homo sapiens
  source 1..2420: mol_type = other RNA
tgccctgcctgttttctcctttttcatttctgcccctatcaaaacttcttttctgccaggtgcagtggaccaacatctgtagttccggctgctcaggaaggtgaagtgggaggatcacttgagcccaggaatttgagtccagcctgggcaacacagcaagacctcattgctttaaaaaaaaaaagtagggctcagtggctcatgcctgtaatcccagctacgtaagaggctcaggcaggaggattacttgagcccaggagttcagggctgcagtgagctgtgattgtgccactgcactccaccctaggtgacagaacaagaccccatctcttaaaaacaaaccaaccaaaaaacacaggtttcgtctcagagaagcggggtgggctctacttagtagtagagtctcttaaaacaatcaacagtagtgtaatttatcaataatcagatagcagacatccctctcagagatctatatattttcagccacaaagcttaaaatctcaaatgtcaacgagtaggatttcaggcaaaataaaagtagaaaataaaaatcagaatgtagatccatgttgggagaggaggttaactttccaggtaattcatactgagattgtttacacagctcctgcgggtccggctttctgtggctttctttagctaaggccagaaattcaaaaaaatcccaatggttatggagatccctcctcacccatccatccacccaatgagaaagaagaatttgtggagggcaggggatatcacaagagaaaatggcacaccagggtgtaatgtctcaaataaaaggcttactttacacttaatactagtatattactgttcataataatatatcgtaaaattatcatgttataaaaatatataataagatcttataagaaactctgaatggattgacgcttgataattctcttaagtagaacacaatgaaacagtagtggctggctaagttccatcaattttttttaattctttttgactttttctcgtggtcttctgttatcctttctgcaggtcgcttcttcaaccccttcattttcctggtttgtagtttgcttaggtcttgcttctgcatatgaatccttccataagttgtaccaaaagtatcatgggaaatatttttcttcttctttggcttgagagcttttggcattttcatagataatttataaaggtcatccgatgccaggtgtgtcctcctcagaaccagatccaatgagggtcccatctcttccaattcaatccgtggtgttctgcaaccagatttcttcaacagcaacttatagcttcgaaagtaaatcttcccattcagtgcagtgaagtgcagaacatactctaatccagccaggcggatatttgatactgtggggcctctgaagaaatcaataagaagactttttagtcttctataatcttctgttacatcgaaatcatcgccagcaaatatcagcatgggttttgttccctcaggacatttactgttcttaatgtcttttagagagacaaaattctcaatacctaattcaatcatatccagcacatggtagtcatacatacgacctattactagattatttggccgcttcttattatgggagccaaacatgaataaagaacaatctgacttctttgaaaagaattccttcaggccaggcacggtggctcacacctgtaatcccagcacttgggacgccgaggcgagttgattacttgagatcaggagtttgagaccagcctggccaacaaggtaagaccgtatctctactaaaaatacaaaagacagccaggtgtgaaggcacacgcctgtaatcccagctaccttagtggctgaggcacgagaatcgcttgaacccagaaggcagaggttgcagtgagctgagaatgcgacactgcactccaacctggggaacagagtaagactctgtctaaaaaaaacaaaacaaaacgaaacaaaaaactctaacagtttttttcttccagtggaagttaatgaagacttaatgaaccagaaagaaaaatacagaggaaaggtatttccagctttttacttcaagtttcctgatttggggtacttagggaaaagatgtgcatttcaagactaagaatacatgaaaactattcagttaataaataaaatgaaaccatttattttgttatgctgtcattttggaatagcacaccaagtgtttcatttgctgaacaaattccttttactcgcaggatatcactactatcattgcatacattcaaaacacacgaggcccagtaaggtggctcatgccagtaatcccagcactgtgggaggctgaggcagacggatcacctgaggtcacctgatgtcaggagtttgagaccagcctggccaacatggtgacaccctgtctctactaaaaataaaaaaa

SEQ ID NO: 18882 - RNA, 3252 nt, Homo sapiens
  source 1..3252: mol_type = other RNA
tgcccttctctcctcctgcctcacgccctttcctgctcctttaaatagcagacacactactctggcgcccccacttccacaaccagaaaatccagcccaagaactactccctaaatataatgcccatagtgatgaaggtgggggtttgaccctttaccccagtattagtcccctcctcacattttcactgagaatggggatacattccatcaataatttgagatgtttctttggaggagtgggggagagggcctccagatgcctgaagaggaatggagggaccatccaaatattcctccccctacttctccccagaaggatggtgtccccaaagctgggctggtaggggcaggggcagggggaagggaagaaagacaaagacaaggaacaagacagagctgggagtgacagccaccaaaagaaagcaaagcaaagagctggagggaaaggaaagagttgaggaaagggaagatcccaaaggaagggaagataggcggagagagtgaagggaaacactgcaggggacaggggcagagaggaggactcctctccagattcctctagcccagctttgtggggacagatggcttctgagcctttcagccacagaaacgattgacatgcttctctccccaacccctagaagatctatgcaacttctgataggactccaactcccttacactgctggaaactggtgacagtttcccaaacaggatatgggggtggggtgggaggtaaagggtcatgttaggaggtcggaggtcaggaccagagggcttagggattgcaaagagcacctctagatacaggtggtaattctccctctcccttttacccaccccctcctcggaagaaggggtggagtgacacacagcgggggaggtgggcagagggcgtcagaatgccttagtggccacctctggcaaaacaaaagtttctcttagctgcttccagatttaagggtgtgttgaggtatcagagttgtaactctagtaaaattttcagtctggccccctcccaatctttccaggacagggtgaccagaggctctgaaagtggcgcaccctccagccaccactgcctccctccccccttccccagcgagcgagtatctctaagcaccttgcccctcaaatcaccgctttccaaaaggctttagtggaaaacaggtccagggtgggcccagtggagtgggccccggaggcatggggcacggggcttaggagaatattcggatggcttgcgtggctgtgatgtggcagacgggacactctgggtccgtcctctcgcagatgcgtactgcacactccatgcagaacaggttgtgtccgcagggcacaagggcggcagtcacttcgctctcaaagcagaccatgcaatcccgcccgccgccggggctccgcaggccgcccccaccaagtttagagaagccctggagcggctctcccggggggcgcctcgggagtccggccagctcgggtcccgcggaagtggcaggggagcggtgtgcgcccgggggcccagcgcgggccttggcggaagaggaggaggaggaggaggcagaggagaagagcacggaggtgggcgtggcgttctcctggcccgcccacagcggggggctagtctcggccacgccgtagtacacatcctgcttgcccacgccatagcccggaaagaggtacccgccgtagccaaagtccccgccctgctcacccaggcgtggggcctcaaagccagagtccactccgcactcgccgatgcagcccaggctgttctgccggaaggtggagaggggcttgcagccgggctggtgcacccgccaggcgtcggagtagcggctatcgattgctgcgtcggggctccccgccaggaagtcgttttcattgttgtactcgaggatcttgccagtgcgcaccgcgatgtgcgtctcgatctcctcgcgcgcacgctccacgttgcctggggcacccgtgatctcgaacacggggtcgcggtcacggcttggtgtgataatgtatgtgttggtttgctgctggatgcgcttgatggttgcccctttggggcccaccaccagccccaccacgcggtagggcacccgcacacggatggtcacctggccgggcagagcaggagccacaccaaaggcggcgcctgacttgttgcgggaggcacggatcatggagaagtgctccgctgctgagatgatttcccgccgggctgtggccacgtcctcccgtcgccctgtcaccatgaacactggttcctcgcccctcaccggtgtcttgatgtaggtgttggtcttggccctcaaggccttaatcttgcagccttgcctgcccacgatctcggccacgtgctcggaggtgggcacgggaacacactccgtggtgttgctgctgcccttcaggcgcagctcggcctctttgtagagagcgcagagcttggcgtcgctcgcccctttgggggcggtggggggctggggcgtctgcgctgcgggggccgccgtcggggcggccgggggcgccgcgggcggcggcggcggggccggctgcgggggggcggccggctgcgcgggggcgccgccccccccacctcccccgtcctcgcccgccgtgggggcggggggctcccccaaacccaggaggcagagttgatcgagagccagctgaagggcgcgctcgtcttccagcagccctcggtccttagcgcttcccccgaaacatcctagttctccaaagcccccatttctttccattattccagataccactagactaggcatggcgaaacaaaagctgggggagagagagagggagagagagagagagaggtggtggaagggaaaagaggagagaggaggggaggggagaggagaggagggggtgtgtggggaggggggaacaaagaactggggaggggggaagaaagcgagatagaaagatagaccctccccctaagcccccctccccaaacaccctgtaacccgactcccctcgccccagcccccggggtgggggtggggggaaagagaagcaaaaccaagaaagcagatctcctctcctctccgggggtgacggggggcggggggctgcaggatctctgcccccacccctcccgcctcggacctgggagtctctagcccccgctgtccaggcgcccccgttaggctcccgcaccgagccccagtccgggagcggcgctcagtggcccccaatagagcccagccccttccagcgctcaaactctttt

SEQ ID NO: 18883 - RNA, 6329 nt, Homo sapiens
  source 1..6329: mol_type = other RNA
tgcccttctctcctcctgcctgccttgcgatggaaataagctcagaaacctctccacttcccagctcagccagccacagagcagcacattggttcaaatgttacccttttctctggcacatccaagcacagtagctcaaccagacatgaacctactgcccaccaaatctgagctcttgaatacacattttctccagtcagatattggtcaaagttttcagccaacttttatccacagccaaagaaaatggcctttcctttctaatagcctgtagatttgtttggaccacatgtctgtttctgtagcatttggtgcatgtcctcaagcctggagctaaatgtgccacattctgtgcaagggaagaagaaatggcaggatggctggacacctctcccagcaattctacaccaagacaaaataaaactggaaacattagctctttgaatgctcccctctccttgttgaaaatccctcttaaggtgctttatccaaagacttttatggaaataaattttgtgttggaaactcactatctgctgtagaggaaacatcgtgtaaagcaggccatcaactatgttttagtattgacatttcaaaaaggcctcatagctcccatgccaccatcccacgcccatccagtccacagtctccattcagccaccaaagggattttcctaaaatgcaattctgatcatgactctatcctgatttaaaggctccagtggctccaaaccccttccatgacaagtctagctcctccacacttcctaccagtttccttaggattcagccctgcctacctatgaagggacccctcaacccctgagcttccacatcatgctctggcaatgccacgttgctcagcggaacccatcatggcatttcatgcgtccacacctttgcacattcttccctcattgtggcatgccctgccaatcctttcattctactggaaatttactctttgttttaaaaccttagcagccattgcttctctcagggtttctctggtccccaagatagttaattgatgctttcttatgccaccttggtacccttgcctgttttgcaatttgtctatacacctcctatgctcatgaacttcttgagggcaggaactatgcctatcctcatgcctggcccttgacccaagctcaatgcatgtttttggaatgcatgaggaatgaaccaactgacaggttcatctatcaatagaaagtgggcccatggcataaattcccagaataatgctgcagcaagactccacccaatgaggcctaagtgaggcctcattgtcaagggaatagagtgtgttgaatgcagaggcaatcaacatcacccccgaagtagaacaactcgcacacaaaaggctgcatcagaggtcgtgttcaccattctcacaacatcgtttgccacttattattctagtcataatgatggctctctttcaacgtcagcataatgcctggtgctcagtggatccttaacaaataccatgtaaggataaatgaataagtgtgaaatctactttttaaaagaaggcatcaagggattggcttttaaaggcatttcccatatgacagatttttctgaggcatgagtgggttgtccctcctaaaatttgacccaatcaggaagtagaacagagatggagcctggggtagcagttaggaatctgcactagagagacacagtgtcaggtttaccttggtcctaggtcagtttccttccttctcaagaaatagccaactatggatggtatttcccgccccaaccagaaggctcttgcctctcctttgtcagaggcacacagtagcatcaccacagtccacattgaccaggaacttcacgtgcagtgatgaggatgagcacagggtgttccctacctttgcttcacgtgctaacattatgcaatggagaacagtcatagagacaaatcctggatgaaaaccaccacccctggggattaaagttgtctgttcaccatagctgttaagagcaagggctctggactcagactgacctggattcaaatccaggatccagatctttctagccaagtcagctgggacaagtcaattatcattttagggggtcaatttcctcacccacaaaatgggaatgatcttacccccctcaaaggattactgtgagggttaaagaatgtaatgtatgtgaagcctgcacagtgtctatagatagcaagtgctcaaaagtggaaaactatgattaagaactttcaaaaatattttcacgatagtcagatcaaaaggaaaaatattctttcaagacacggtgctttcaagagaatggattgtctaatttttaggagccaacaaatgctcattaatcaatgccccacggaagaacatgagaagacagtgttggcatttaaaacaataactgtggccattaccaggccccaggatggacagatagggacaaggacagggatacccagcatttctctgagagctggtgcaagaggattaatcctgaagggctcatttctgattctcctctgctggacaaagaatgactgagttggaacctcagagggtgcaagtcaaggtgccaagagtaagatgccagtttcggtctgtaagcaagtgtttctgggggtgagggaaggtcaggggaaacctgaccactggacaggagtgaggcaggtacagtgcattgctccaggtgtcatgcaaagctagaaagtcagcatttcctctgttgttttgatcctccttatacaacccaaagccaacagaggatttcaacttccccaaatttctgccctgagcattaaacaactttttcctatgctaaatttggttttagttttgaagtgcctgagatgcacaattcaaaggggtcaagttcctggcctcttatgttgatgaaaccatccccaatcctcagcttacatggcttgcccctatgcctaccacctcttatagctcttccatccatcattcaagaggttccatgaagaaagctcagggttaatgtttggggtagtacaagctaagccatcagcccttgggaacaaagattactttctgttggaggggtcaatttggctagtcactttgagcagcagggcagggacccaaagtggaaaagagaagagatttttaaatgtagagatagctccatccacaggagattggattcctgggaagaaatggaccttactcaggggaagccttgacctctgatttagtctgagcctgtgagagctcacggcccatttctggccttcttgccctaggctcagattggtggacagcatccaaacaaaggcagcccacaactaggcagtgttgtgtagtagaaggagcactggactggaagtcaggagacctgaattcgagtgcaggctctgccgctaactagctgtgtgaccttgggcaagtcacctgatttctcttgggcaactgtaaaacgaagggttggtcgggtgatctctaagttccccttccgaatgtggtccagggtcctactctatccctccttagccctgtgcttgcagggacagagatgggagaagggaaggggaggagagagaggaggcaggagggagcccaagggtgtcatgaatcaggactccactttctccttctttttgctctttttcaggaaggagggggttcggaatttctttttcttctttgagggagacttggaaggtgagccctctggggacatggggccgctggtgaccgactcggttttgtccttagaggtatcaacatccgtgtcagcactggtggtcatctggctcaggcctttgctgaggatttcctctgccgtctgctcctcctccctcccgttgaccaccaccccttccggctgggttgtttcgggctctgtggtggcggctttgcttgtttctgtcttcttagtaccttcctctaaagacttggaaggagagactaaagggctctttgtctctgcctccttcgctgggctctgcactggagaagcaggtgcagactttgcaggtgagccaggctcttctggggcagtttctttctctccaatatgttactccagatgtggagggcaacgctgaagaactcgcacacggccggaccagagcctggctctcgttcctgtcctgtctcatcaagttctagtttcttcctctccacctctttcttgtactcctccaactcctggtcagtgagttggctgaaggggttgggcaccgtctcctctgaatcgtctttggtatcctcgtctcccttggacatcagctggctctctgtagacgggcttcggctcttctcggcaatgacgctcgccaggagctgggactgaggccccgctgacttcacatcttgtcggttttgttctcgaatcttgttcctcatctccagtacttcctgggggtcagtatagagaggcacaaattggtttgggttttcgatgcgaatcggcatgccactgctggatttctccacctcgtcagccttcatccacgtggtcttgggtcgggggctgcccatgctcctctggacctcatcggccacattgacccgcaggtaggtgttgggcgtattgagccagcgggtcttctccttctgctgcttctgggcatgctgtcgcagggcgggcaccggggcaccgtcctcctcaaacacgaaggctgtgaccgtggctggaatctccacctcacttttgtgtttggttttctcttgaacaaaggggtggcgatacgtgtaacctgttctgtagcccaggttgtccagcatcctcatgagggcctcaaactcatgctcccccagccgactcttctgcataggcccaaaggtgctcccggcccactgcacggagcccacctcatggggccggtgcttctcctgctccaggaggatgaggttctccactcccccggcactggacagagccgacacctgtatctcacatgcagcctgcaggtggaagatcttgtaaaatgcctcctctaccgtgtcacccagagcaaccactccatggtttcttagcaccaggatcttgcaggtgggtccaaggcacttctgcaggttgatccgatcggcttcctgctccatttccccattgaagtcataataggccatgtcccccaccagcagggcattgtgggagacaggcaggaggccccacttcatggccgacaccgctgctgtggccggtgtgtgcaggtggatgatgcagcgcacgtcgggcctcgctgcatagatggccgagtgcagacagaagcctgtggtgtccactgggaagcagctgctgcccttctccaccacctctcccagaatgttcaccttgatcaggctggacgctgtgacttcactgcaagaaactcccttagggctgatcaggaagtggtcctgctccttgctgactctcaacgtgacataggtgtcactcagctgggcccagccatagaggtccaggagtcggtagacactgctgatcttgcaccgcatgagccgctcccctttggccaggttcagggagtcagctgtgtggaggtcattgataggcgtcatcatggagacattcatggaagatgtcgggaagactgcgtgggaggtgctggccatgaagtccgcgatctgtcgcagggcccagatgttggaggagttgttccccttcttcatctgctcctggatgaggccttccagctcctccctgaaagagggactctgcaggatcatggtgacgcgcttcttctgctccatcaggttgaagtcctgccgcaggtccgccgcccggttgcgaaggcgcatgtactcggggtcgtcctctgagaagcggtcaaagtaaggctgcccctgcgggggcggcggcgaggcagcctcggggaccgtctcttcgctcattttcccggtgggtttgcaattcgctcctggaactcgggaggctggcccagccctgtccaaggctccttctgttcactgctcagtctgcaccccctagctccactctcaagggtgccggccacatctacacaacctcaaacatccaggtggaaactcctgcgcggcatcttagctatctccggtcggccactgcgggttggttttgttattttatgggtttggggggtggggtgcgcttaaaaaatccacccagctaatctgcagggcagcgttttctgcccatgctgcagcccgcgctcgtcagagctgctgggagatcccccagcagtgcagcggctccgcggcggcggggatgactggccaccgacgccgcagttccttgacaaaaggctcgggttcccgctagtccctcacagccctgccgtcagaattaaagccatttcccgcacgaggctgggaggaaatgag

SEQ ID NO: 18884 - RNA, 6027 nt, Homo sapiens
  source 1..6027: mol_type = other RNA
tgcccttctctcctcctgcctgccttgcgatggaaataagctcagaaacctctccacttcccagctcagccagccacagagcagcacattggttcaaatgttacccttttctctggcacatccaagcacagtagctcaaccagacatgaacctactgcccaccaaatctgagctcttgaatacacattttctccagtcagatattggtcaaagttttcagccaacttttatccacagccaaagaaaatggcctttcctttctaatagcctgtagatttgtttggaccacatgtctgtttctgtagcatttggtgcatgtcctcaagcctggagctaaatgtgccacattctgtgcaagggaagaagaaatggcaggatggctggacacctctcccagcaattctacaccaagacaaaataaaactggaaacattagctctttgaatgctcccctctccttgttgaaaatccctcttaaggtgctttatccaaagacttttatggaaataaattttgtgttggaaactcactatctgctgtagaggaaacatcgtgtaaagcaggccatcaactatgttttagtattgacatttcaaaaaggcctcatagctcccatgccaccatcccacgcccatccagtccacagtctccattcagccaccaaagggattttcctaaaatgcaattctgatcatgactctatcctgatttaaaggctccagtggctccaaaccccttccatgacaagtctagctcctccacacttcctaccagtttccttaggattcagccctgcctacctatgaagggacccctcaacccctgagcttccacatcatgctctggcaatgccacgttgctcagcggaacccatcatggcatttcatgcgtccacacctttgcacattcttccctcattgtggcatgccctgccaatcctttcattctactggaaatttactctttgttttaaaaccttagcagccattgcttctctcagggtttctctggtccccaagatagttaattgatgctttcttatgccaccttggtacccttgcctgttttgcaatttgtctatacacctcctatgctcatgaacttcttgagggcaggaactatgcctatcctcatgcctggcccttgacccaagctcaatgcatgtttttggaatgcatgaggaatgaaccaactgacaggttcatctatcaatagaaagtgggcccatggcataaattcccagaataatgctgcagcaagactccacccaatgaggcctaagtgaggcctcattgtcaagggaatagagtgtgttgaatgcagaggcaatcaacatcacccccgaagtagaacaactcgcacacaaaaggctgcatcagaggtcgtgttcaccattctcacaacatcgtttgccacttattattctagtcataatgatggctctctttcaacgtcagcataatgcctggtgctcagtggatccttaacaaataccatgtaaggataaatgaataagtgtgaaatctactttttaaaagaaggcatcaagggattggcttttaaaggcatttcccatatgacagatttttctgaggcatgagtgggttgtccctcctaaaatttgacccaatcaggaagtagaacagagatggagcctggggtagcagttaggaatctgcactagagagacacagtgtcaggtttaccttggtcctaggtcagtttccttccttctcaagaaatagccaactatggatggtatttcccgccccaaccagaaggctcttgcctctcctttgtcagaggcacacagtagcatcaccacagtccacattgaccaggaacttcacgtgcagtgatgaggatgagcacagggtgttccctacctttgcttcacgtgctaacattatgcaatggagaacagtcatagagacaaatcctggatgaaaaccaccacccctggggattaaagttgtctgttcaccatagctgttaagagcaagggctctggactcagactgacctggattcaaatccaggatccagatctttctagccaagtcagctgggacaagtcaattatcattttagggggtcaatttcctcacccacaaaatgggaatgatcttacccccctcaaaggattactgtgagggttaaagaatgtaatgtatgtgaagcctgcacagtgtctatagatagcaagtgctcaaaagtggaaaactatgattaagaactttcaaaaatattttcacgatagtcagatcaaaaggaaaaatattctttcaagacacggtgctttcaagagaatggattgtctaatttttaggagccaacaaatgctcattaatcaatgccccacggaagaacatgagaagacagtgttggcatttaaaacaataactgtggccattaccaggccccaggatggacagatagggacaaggacagggatacccagcatttctctgagagctggtgcaagaggattaatcctgaagggctcatttctgattctcctctgctggacaaagaatgactgagttggaacctcagagggtgcaagtcaaggtgccaagagtaagatgccagtttcggtctgtaagcaagtgtttctgggggtgagggaaggtcaggggaaacctgaccactggacaggagtgaggcaggtacagtgcattgctccaggtgtcatgcaaagctagaaagtcagcatttcctctgttgttttgatcctccttatacaacccaaagccaacagaggatttcaacttccccaaatttctgccctgagcattaaacaactttttcctatgctaaatttggttttagttttgaagtgcctgagatgcacaattcaaaggggtcaagttcctggcctcttatgttgatgaaaccatccccaatcctcagcttacatggcttgcccctatgcctaccacctcttatagctcttccatccatcattcaagaggttccatgaagaaagctcagggttaatgtttggggtagtacaagctaagccatcagcccttgggaacaaagattactttctgttggaggggtcaatttggctagtcactttgagcagcagggcagggacccaaagtggaaaagagaagagatttttaaatgtagagatagctccatccacaggagattggattcctgggaagaaatggaccttactcaggggaagccttgacctctgatttagtctgagcctgtgagagctcacggcccatttctggccttcttgccctaggctcagattggtggacagcatccaaacaaaggcagcccacaactaggcagtgttgtgtagtagaaggagcactggactggaagtcaggagacctgaattcgagtgcaggctctgccgctaactagctgtgtgaccttgggcaagtcacctgatttctcttgggcaactgtaaaacgaagggttggtcgggtgatctctaagttccccttccgaatgtggtccagggtcctactctatccctccttagccctgtgcttgcagggacagagatgggagaagggaaggggaggagagagaggaggcaggagggagcccaagggtgtcatgaatcaggactccactttctccttctttttgctctttttcaggaaggagggggttcggaatttctttttcttctttgagggagacttggaaggtgagccctctggggacatggggccgctggtgaccgactcggttttgtccttagaggtatcaacatccgtgtcagcactggtggtcatctggctcaggcctttgctgaggatttcctctgccgtctgctcctcctccctcccgttgaccaccaccccttccggctgggttgtttcgggctctgtggtggcggctttgcttgtttctgtcttcttagtaccttcctctaaagacttggaaggagagactaaagggctctttgtctctgcctccttcgctgggctctgcactggagaagcaggtgcagactttgcaggtgagccaggctcttctggggcagtttctttctctccatcaagttctagtttcttcctctccacctctttcttgtactcctccaactcctggtcagtgagttggctgaaggggttgggcaccgtctcctctgaatcgtctttggtatcctcgtctcccttggacatcagctggctctctgtagacgggcttcggctcttctcggcaatgacgctcgccaggagctgggactgaggccccgctgacttcacatcttgtcggttttgttctcgaatcttgttcctcatctccagtacttcctgggggtcagtatagagaggcacaaattggtttgggttttcgatgcgaatcggcatgccactgctggatttctccacctcgtcagccttcatccacgtggtcttgggtcgggggctgcccatgctcctctggacctcatcggccacattgacccgcaggtaggtgttgggcgtattgagccagcgggtcttctccttctgctgcttctgggcatgctgtcgcagggcgggcaccggggcaccgtcctcctcaaacacgaaggctgtgaccgtggctggaatctccacctcacttttgtgtttggttttctcttgaacaaaggggtggcgatacgtgtaacctgttctgtagcccaggttgtccagcatcctcatgagggcctcaaactcatgctcccccagccgactcttctgcataggcccaaaggtgctcccggcccactgcacggagcccacctcatggggccggtgcttctcctgctccaggaggatgaggttctccactcccccggcactggacagagccgacacctgtatctcacatgcagcctgcaggtggaagatcttgtaaaatgcctcctctaccgtgtcacccagagcaaccactccatggtttcttagcaccaggatcttgcaggtgggtccaaggcacttctgcaggttgatccgatcggcttcctgctccatttccccattgaagtcataataggccatgtcccccaccagcagggcattgtgggagacaggcaggaggccccacttcatggccgacaccgctgctgtggccggtgtgtgcaggtggatgatgcagcgcacgtcgggcctcgctgcatagatggccgagtgcagacagaagcctgtggtgtccactgggaagcagctgctgcccttctccaccacctctcccagaatgttcaccttgatcaggctggacgctgtgacttcactgcaagaaactcccttagggctgatcaggaagtggtcctgctccttgctgactctcaacgtgacataggtgtcactcagctgggcccagccatagaggtccaggagtcggtagacactgctgatcttgcaccgcatgagccgctcccctttggccaggttcagggagtcagctgtgtggaggtcattgataggcgtcatcatggagacattcatggaagatgtcgggaagactgcgtgggaggtgctggccatgaagtccgcgatctgtcgcagggcccagatgttggaggagttgttccccttcttcatctgctcctggatgaggccttccagctcctccctgaaagagggactctgcaggatcatggtgacgcgcttcttctgctccatcaggttgaagtcctgccgcaggtccgccgcccggttgcgaaggcgcatgtactcggggtcgtcctctgagaagcggtcaaagtaaggctgcccctgcgggggcggcggcgaggcagcctcggggaccgtctcttcgctcattttcccggtgggtttgcaattcgctcctggaactcgggaggctggcccagccctgtccaaggctccttctgttcactgctcagtctgcaccccctagctccactctcaagggtgccggccacatctacacaacctcaaacatccaggtggaaacgatccctaaatgagactcccacaagtgagagaggagatggtcagggctgagctgctgctacttttacagaataaatgaagacagttgaataagggact

SEQ ID NO: 18885 - RNA, 6243 nt, Homo sapiens
  source 1..6243: mol_type = other RNA
tgcccttctctcctcctgcctgccttgcgatggaaataagctcagaaacctctccacttcccagctcagccagccacagagcagcacattggttcaaatgttacccttttctctggcacatccaagcacagtagctcaaccagacatgaacctactgcccaccaaatctgagctcttgaatacacattttctccagtcagatattggtcaaagttttcagccaacttttatccacagccaaagaaaatggcctttcctttctaatagcctgtagatttgtttggaccacatgtctgtttctgtagcatttggtgcatgtcctcaagcctggagctaaatgtgccacattctgtgcaagggaagaagaaatggcaggatggctggacacctctcccagcaattctacaccaagacaaaataaaactggaaacattagctctttgaatgctcccctctccttgttgaaaatccctcttaaggtgctttatccaaagacttttatggaaataaattttgtgttggaaactcactatctgctgtagaggaaacatcgtgtaaagcaggccatcaactatgttttagtattgacatttcaaaaaggcctcatagctcccatgccaccatcccacgcccatccagtccacagtctccattcagccaccaaagggattttcctaaaatgcaattctgatcatgactctatcctgatttaaaggctccagtggctccaaaccccttccatgacaagtctagctcctccacacttcctaccagtttccttaggattcagccctgcctacctatgaagggacccctcaacccctgagcttccacatcatgctctggcaatgccacgttgctcagcggaacccatcatggcatttcatgcgtccacacctttgcacattcttccctcattgtggcatgccctgccaatcctttcattctactggaaatttactctttgttttaaaaccttagcagccattgcttctctcagggtttctctggtccccaagatagttaattgatgctttcttatgccaccttggtacccttgcctgttttgcaatttgtctatacacctcctatgctcatgaacttcttgagggcaggaactatgcctatcctcatgcctggcccttgacccaagctcaatgcatgtttttggaatgcatgaggaatgaaccaactgacaggttcatctatcaatagaaagtgggcccatggcataaattcccagaataatgctgcagcaagactccacccaatgaggcctaagtgaggcctcattgtcaagggaatagagtgtgttgaatgcagaggcaatcaacatcacccccgaagtagaacaactcgcacacaaaaggctgcatcagaggtcgtgttcaccattctcacaacatcgtttgccacttattattctagtcataatgatggctctctttcaacgtcagcataatgcctggtgctcagtggatccttaacaaataccatgtaaggataaatgaataagtgtgaaatctactttttaaaagaaggcatcaagggattggcttttaaaggcatttcccatatgacagatttttctgaggcatgagtgggttgtccctcctaaaatttgacccaatcaggaagtagaacagagatggagcctggggtagcagttaggaatctgcactagagagacacagtgtcaggtttaccttggtcctaggtcagtttccttccttctcaagaaatagccaactatggatggtatttcccgccccaaccagaaggctcttgcctctcctttgtcagaggcacacagtagcatcaccacagtccacattgaccaggaacttcacgtgcagtgatgaggatgagcacagggtgttccctacctttgcttcacgtgctaacattatgcaatggagaacagtcatagagacaaatcctggatgaaaaccaccacccctggggattaaagttgtctgttcaccatagctgttaagagcaagggctctggactcagactgacctggattcaaatccaggatccagatctttctagccaagtcagctgggacaagtcaattatcattttagggggtcaatttcctcacccacaaaatgggaatgatcttacccccctcaaaggattactgtgagggttaaagaatgtaatgtatgtgaagcctgcacagtgtctatagatagcaagtgctcaaaagtggaaaactatgattaagaactttcaaaaatattttcacgatagtcagatcaaaaggaaaaatattctttcaagacacggtgctttcaagagaatggattgtctaatttttaggagccaacaaatgctcattaatcaatgccccacggaagaacatgagaagacagtgttggcatttaaaacaataactgtggccattaccaggccccaggatggacagatagggacaaggacagggatacccagcatttctctgagagctggtgcaagaggattaatcctgaagggctcatttctgattctcctctgctggacaaagaatgactgagttggaacctcagagggtgcaagtcaaggtgccaagagtaagatgccagtttcggtctgtaagcaagtgtttctgggggtgagggaaggtcaggggaaacctgaccactggacaggagtgaggcaggtacagtgcattgctccaggtgtcatgcaaagctagaaagtcagcatttcctctgttgttttgatcctccttatacaacccaaagccaacagaggatttcaacttccccaaatttctgccctgagcattaaacaactttttcctatgctaaatttggttttagttttgaagtgcctgagatgcacaattcaaaggggtcaagttcctggcctcttatgttgatgaaaccatccccaatcctcagcttacatggcttgcccctatgcctaccacctcttatagctcttccatccatcattcaagaggttccatgaagaaagctcagggttaatgtttggggtagtacaagctaagccatcagcccttgggaacaaagattactttctgttggaggggtcaatttggctagtcactttgagcagcagggcagggacccaaagtggaaaagagaagagatttttaaatgtagagatagctccatccacaggagattggattcctgggaagaaatggaccttactcaggggaagccttgacctctgatttagtctgagcctgtgagagctcacggcccatttctggccttcttgccctaggctcagattggtggacagcatccaaacaaaggcagcccacaactaggcagtgttgtgtagtagaaggagcactggactggaagtcaggagacctgaattcgagtgcaggctctgccgctaactagctgtgtgaccttgggcaagtcacctgatttctcttgggcaactgtaaaacgaagggttggtcgggtgatctctaagttccccttccgaatgtggtccagggtcctactctatccctccttagccctgtgcttgcagggacagagatgggagaagggaaggggaggagagagaggaggcaggagggagcccaagggtgtcatgaatcaggactccactttctccttctttttgctctttttcaggaaggagggggttcggaatttctttttcttctttgagggagacttggaaggtgagccctctggggacatggggccgctggtgaccgactcggttttgtccttagaggtatcaacatccgtgtcagcactggtggtcatctggctcaggcctttgctgaggatttcctctgccgtctgctcctcctccctcccgttgaccaccaccccttccggctgggttgtttcgggctctgtggtggcggctttgcttgtttctgtcttcttagtaccttcctctaaagacttggaaggagagactaaagggctctttgtctctgcctccttcgctgggctctgcactggagaagcaggtgcagactttgcaggtgagccaggctcttctggggcagtttctttctctccatcaagttctagtttcttcctctccacctctttcttgtactcctccaactcctggtcagtgagttggctgaaggggttgggcaccgtctcctctgaatcgtctttggtatcctcgtctcccttggacatcagctggctctctgtagacgggcttcggctcttctcggcaatgacgctcgccaggagctgggactgaggccccgctgacttcacatcttgtcggttttgttctcgaatcttgttcctcatctccagtacttcctgggggtcagtatagagaggcacaaattggtttgggttttcgatgcgaatcggcatgccactgctggatttctccacctcgtcagccttcatccacgtggtcttgggtcgggggctgcccatgctcctctggacctcatcggccacattgacccgcaggtaggtgttgggcgtattgagccagcgggtcttctccttctgctgcttctgggcatgctgtcgcagggcgggcaccggggcaccgtcctcctcaaacacgaaggctgtgaccgtggctggaatctccacctcacttttgtgtttggttttctcttgaacaaaggggtggcgatacgtgtaacctgttctgtagcccaggttgtccagcatcctcatgagggcctcaaactcatgctcccccagccgactcttctgcataggcccaaaggtgctcccggcccactgcacggagcccacctcatggggccggtgcttctcctgctccaggaggatgaggttctccactcccccggcactggacagagccgacacctgtatctcacatgcagcctgcaggtggaagatcttgtaaaatgcctcctctaccgtgtcacccagagcaaccactccatggtttcttagcaccaggatcttgcaggtgggtccaaggcacttctgcaggttgatccgatcggcttcctgctccatttccccattgaagtcataataggccatgtcccccaccagcagggcattgtgggagacaggcaggaggccccacttcatggccgacaccgctgctgtggccggtgtgtgcaggtggatgatgcagcgcacgtcgggcctcgctgcatagatggccgagtgcagacagaagcctgtggtgtccactgggaagcagctgctgcccttctccaccacctctcccagaatgttcaccttgatcaggctggacgctgtgacttcactgcaagaaactcccttagggctgatcaggaagtggtcctgctccttgctgactctcaacgtgacataggtgtcactcagctgggcccagccatagaggtccaggagtcggtagacactgctgatcttgcaccgcatgagccgctcccctttggccaggttcagggagtcagctgtgtggaggtcattgataggcgtcatcatggagacattcatggaagatgtcgggaagactgcgtgggaggtgctggccatgaagtccgcgatctgtcgcagggcccagatgttggaggagttgttccccttcttcatctgctcctggatgaggccttccagctcctccctgaaagagggactctgcaggatcatggtgacgcgcttcttctgctccatcaggttgaagtcctgccgcaggtccgccgcccggttgcgaaggcgcatgtactcggggtcgtcctctgagaagcggtcaaagtaaggctgcccctgcgggggcggcggcgaggcagcctcggggaccgtctcttcgctcattttcccggtgggtttgcaattcgctcctggaactcgggaggctggcccagccctgtccaaggctccttctgttcactgctcagtctgcaccccctagctccactctcaagggtgccggccacatctacacaacctcaaacatccaggtggaaactcctgcgcggcatcttagctatctccggtcggccactgcgggttggttttgttattttatgggtttggggggtggggtgcgcttaaaaaatccacccagctaatctgcagggcagcgttttctgcccatgctgcagcccgcgctcgtcagagctgctgggagatcccccagcagtgcagcggctccgcggcggcggggatgactggccaccgacgccgcagttccttgacaaaaggctcgggttcccgctagtccctcacagccctgccgtcagaattaaagccatttcccgcacgaggctgggaggaaatgag

SEQ ID NO: 18886 - RNA, 6040 nt, Homo sapiens
  source 1..6040: mol_type = other RNA
tgcccttctctcctcctgcctgccttgcgatggaaataagctcagaaacctctccacttcccagctcagccagccacagagcagcacattggttcaaatgttacccttttctctggcacatccaagcacagtagctcaaccagacatgaacctactgcccaccaaatctgagctcttgaatacacattttctccagtcagatattggtcaaagttttcagccaacttttatccacagccaaagaaaatggcctttcctttctaatagcctgtagatttgtttggaccacatgtctgtttctgtagcatttggtgcatgtcctcaagcctggagctaaatgtgccacattctgtgcaagggaagaagaaatggcaggatggctggacacctctcccagcaattctacaccaagacaaaataaaactggaaacattagctctttgaatgctcccctctccttgttgaaaatccctcttaaggtgctttatccaaagacttttatggaaataaattttgtgttggaaactcactatctgctgtagaggaaacatcgtgtaaagcaggccatcaactatgttttagtattgacatttcaaaaaggcctcatagctcccatgccaccatcccacgcccatccagtccacagtctccattcagccaccaaagggattttcctaaaatgcaattctgatcatgactctatcctgatttaaaggctccagtggctccaaaccccttccatgacaagtctagctcctccacacttcctaccagtttccttaggattcagccctgcctacctatgaagggacccctcaacccctgagcttccacatcatgctctggcaatgccacgttgctcagcggaacccatcatggcatttcatgcgtccacacctttgcacattcttccctcattgtggcatgccctgccaatcctttcattctactggaaatttactctttgttttaaaaccttagcagccattgcttctctcagggtttctctggtccccaagatagttaattgatgctttcttatgccaccttggtacccttgcctgttttgcaatttgtctatacacctcctatgctcatgaacttcttgagggcaggaactatgcctatcctcatgcctggcccttgacccaagctcaatgcatgtttttggaatgcatgaggaatgaaccaactgacaggttcatctatcaatagaaagtgggcccatggcataaattcccagaataatgctgcagcaagactccacccaatgaggcctaagtgaggcctcattgtcaagggaatagagtgtgttgaatgcagaggcaatcaacatcacccccgaagtagaacaactcgcacacaaaaggctgcatcagaggtcgtgttcaccattctcacaacatcgtttgccacttattattctagtcataatgatggctctctttcaacgtcagcataatgcctggtgctcagtggatccttaacaaataccatgtaaggataaatgaataagtgtgaaatctactttttaaaagaaggcatcaagggattggcttttaaaggcatttcccatatgacagatttttctgaggcatgagtgggttgtccctcctaaaatttgacccaatcaggaagtagaacagagatggagcctggggtagcagttaggaatctgcactagagagacacagtgtcaggtttaccttggtcctaggtcagtttccttccttctcaagaaatagccaactatggatggtatttcccgccccaaccagaaggctcttgcctctcctttgtcagaggcacacagtagcatcaccacagtccacattgaccaggaacttcacgtgcagtgatgaggatgagcacagggtgttccctacctttgcttcacgtgctaacattatgcaatggagaacagtcatagagacaaatcctggatgaaaaccaccacccctggggattaaagttgtctgttcaccatagctgttaagagcaagggctctggactcagactgacctggattcaaatccaggatccagatctttctagccaagtcagctgggacaagtcaattatcattttagggggtcaatttcctcacccacaaaatgggaatgatcttacccccctcaaaggattactgtgagggttaaagaatgtaatgtatgtgaagcctgcacagtgtctatagatagcaagtgctcaaaagtggaaaactatgattaagaactttcaaaaatattttcacgatagtcagatcaaaaggaaaaatattctttcaagacacggtgctttcaagagaatggattgtctaatttttaggagccaacaaatgctcattaatcaatgccccacggaagaacatgagaagacagtgttggcatttaaaacaataactgtggccattaccaggccccaggatggacagatagggacaaggacagggatacccagcatttctctgagagctggtgcaagaggattaatcctgaagggctcatttctgattctcctctgctggacaaagaatgactgagttggaacctcagagggtgcaagtcaaggtgccaagagtaagatgccagtttcggtctgtaagcaagtgtttctgggggtgagggaaggtcaggggaaacctgaccactggacaggagtgaggcaggtacagtgcattgctccaggtgtcatgcaaagctagaaagtcagcatttcctctgttgttttgatcctccttatacaacccaaagccaacagaggatttcaacttccccaaatttctgccctgagcattaaacaactttttcctatgctaaatttggttttagttttgaagtgcctgagatgcacaattcaaaggggtcaagttcctggcctcttatgttgatgaaaccatccccaatcctcagcttacatggcttgcccctatgcctaccacctcttatagctcttccatccatcattcaagaggttccatgaagaaagctcagggttaatgtttggggtagtacaagctaagccatcagcccttgggaacaaagattactttctgttggaggggtcaatttggctagtcactttgagcagcagggcagggacccaaagtggaaaagagaagagatttttaaatgtagagatagctccatccacaggagattggattcctgggaagaaatggaccttactcaggggaagccttgacctctgatttagtctgagcctgtgagagctcacggcccatttctggccttcttgccctaggctcagattggtggacagcatccaaacaaaggcagcccacaactaggcagtgttgtgtagtagaaggagcactggactggaagtcaggagacctgaattcgagtgcaggctctgccgctaactagctgtgtgaccttgggcaagtcacctgatttctcttgggcaactgtaaaacgaagggttggtcgggtgatctctaagttccccttccgaatgtggtccagggtcctactctatccctccttagccctgtgcttgcagggacagagatgggagaagggaaggggaggagagagaggaggcaggagggagcccaagggtgtcatgaatcaggactccactttctccttctttttgctctttttcaggaaggagggggttcggaatttctttttcttctttgagggagacttggaaggtgagccctctggggacatggggccgctggtgaccgactcggttttgtccttagaggtatcaacatccgtgtcagcactggtggtcatctggctcaggcctttgctgaggatttcctctgccgtctgctcctcctccctcccgttgaccaccaccccttccggctgggttgtttcgggctctgtggtggcggctttgcttgtttctgtcttcttagtaccttcctctaaagacttggaaggagagactaaagggctctttgtctctgcctccttcgctgggctctgcactggagaagcaggtgcagactttgcaggtgagccaggctcttctggggcagtttctttctctccatcaagttctagtttcttcctctccacctctttcttgtactcctccaactcctggtcagtgagttggctgaaggggttgggcaccgtctcctctgaatcgtctttggtatcctcgtctcccttggacatcagctggctctctgtagacgggcttcggctcttctcggcaatgacgctcgccaggagctgggactgaggccccgctgacttcacatcttgtcggttttgttctcgaatcttgttcctcatctccagtacttcctgggggtcagtatagagaggcacaaattggtttgggttttcgatgcgaatcggcatgccactgctggatttctccacctcgtcagccttcatccacgtggtcttgggtcgggggctgcccatgctcctctggacctcatcggccacattgacccgcaggtaggtgttgggcgtattgagccagcgggtcttctccttctgctgcttctgggcatgctgtcgcagggcgggcaccggggcaccgtcctcctcaaacacgaaggctgtgaccgtggctggaatctccacctcacttttgtgtttggttttctcttgaacaaaggggtggcgatacgtgtaacctgttctgtagcccaggttgtccagcatcctcatgagggcctcaaactcatgctcccccagccgactcttctgcataggcccaaaggtgctcccggcccactgcacggagcccacctcatggggccggtgcttctcctgctccaggaggatgaggttctccactcccccggcactggacagagccgacacctgtatctcacatgcagcctgcaggtggaagatcttgtaaaatgcctcctctaccgtgtcacccagagcaaccactccatggtttcttagcaccaggatcttgcaggtgggtccaaggcacttctgcaggttgatccgatcggcttcctgctccatttccccattgaagtcataataggccatgtcccccaccagcagggcattgtgggagacaggcaggaggccccacttcatggccgacaccgctgctgtggccggtgtgtgcaggtggatgatgcagcgcacgtcgggcctcgctgcatagatggccgagtgcagacagaagcctgtggtgtccactgggaagcagctgctgcccttctccaccacctctcccagaatgttcaccttgatcaggctggacgctgtgacttcactgcaagaaactcccttagggctgatcaggaagtggtcctgctccttgctgactctcaacgtgacataggtgtcactcagctgggcccagccatagaggtccaggagtcggtagacactgctgatcttgcaccgcatgagccgctcccctttggccaggttcagggagtcagctgtgtggaggtcattgataggcgtcatcatggagacattcatggaagatgtcgggaagactgcgtgggaggtgctggccatgaagtccgcgatctgtcgcagggcccagatgttggaggagttgttccccttcttcatctgctcctggatgaggccttccagctcctccctgaaagagggactctgcaggatcatggtgacgcgcttcttctgctccatcaggttgaagtcctgccgcaggtccgccgcccggttgcgaaggcgcatgtactcggggtcgtcctctgagaagcggtcaaagtaaggctgcccctgcgggggcggcggcgaggcagcctcggggaccgtctcttcgctcattttcccggtgggtttgcaattcgctcctggaactcgggaggctggcccagccctgtccaaggctccttctgttcactgctcagtctgcaccccctagctccactctcaagggtgccggccacatctacacaacctcaaacatccaggtggaaactgtcaggcgttacgctccgggcgagggtcccaccatccccaagcaggggccagtgcttgcagccccgatttcctaagagcctcggatgctacatcatcaccagaaaccttt

SEQ ID NO: 18887 - RNA, 3656 nt, Homo sapiens
  source 1..3656: mol_type = other RNA
tgcctactgagctgaaacacagactcaaagctggtttattgttgtcatgactacgagttccacatgcctaaagtcactggtttctgaaaagaatgatgcagtgtctagccttacagctggacatataaaccaaattagtctgccatgcctctacctgctttgtggttattagtgaaaagagcaatatatcacacaatcagtcatgcagcagttaagctctgcacacactgctttttcagatctgtaactcatttttcttccagctccccagaacaataacttgaaatctgcagggaaaaaatcaaagaaattttgacagatattttaaatttttgaatggaagataaaccaaaaagcaatttatagtgtttttttgtactaacaccaccttaattttaaatcacgcaaagagtaacaggatttcataaattctttataaaggagctcaaaacttcactgatttgcaaaagacttaaaaaaaaaaaagagggtgtttcagaaaggagaaccctagtttgcctgctccagatgtgaaatgagagccttgagagctggattctattccttgctctccaagtgattaattgaatgacctaggggaagtaatttaacccagccgtgtaaaaagaaaatatgcatttacccacaagaacagggtgtctaagttggatccacacctgcaccactgacatcactgcctcttctgaagcactcttaagatgccctcccttgcttgtatccctccctccagtctaccctcatttgtctccacctcctgctttaaactcttccaatcttatcaagctcataaatattttagattccctgcctccttcctccacctggttctgttatatctctagtatgtactcaaagaaagctcaaaactgtaaaagattcagtctgtctttgtcatctcactctcctggccccagtccatttggggctcctttttcaaactcttggcatattcatgctgtccacatggctgttgggagtctcactctaaagtatccaacttggacttgccctcactaagcaggtatctgtgtcgtaaaacttccctatattctctctcctttctcctgtcaatggtcagttttcatcatctctccctatttaatacgctttgtatggccagttcatcctaggtggaaacaggtatgaggagtgacagtggaaaccattgctccaatgagcagtcaaaggtagcaagactggaagcagagttgcttcttcggcagggacacataaaattaggggtaaatgagtgggtgctgcccatactacagtataatctcatgttgataataaatttaatatgctaatttgttcccctttgtaggtaatatactcacactttagaggagccatcagcttatattaatagaatgagtatagtgatatagtgatagaaatttcaagtattatgacagccagcgagtgacacctttttgagcctggaaagttgtttcttgggcacttggatcttaggtagttggattgcgtcaagtctacaagtatttgaatccaggtgagccagaattatctgcgactgagaaaaatgcaggatagaagacaattttaaagcactgtgcgattgcatggagtcagccaaaacaggagttcaaaccatatctcatcgtataatctgtaaagtctcttagagaacgttaggtacctgttctttggccagtgggcacagtatagaacaacagatcctttgaggatccctatacatggttgatcatatactattgaggatattttgctagatttatttacatattagaaaaacttttcattaaaatgcacaatgactcatctgatttagatttgtgttagtttttttccccaagtactaagaaacaactttaatttaaataaccactttacgatgcctccaggcaactgcagcacatgtttggttattgatggtcctgtagagctttaaccagttatagaactctatagaatatatatttttttcggcagcttggctttccacacaaaggtaaagatcttgaaaagtgtatacaaagtttttaatatctagttagatgacccattgtatgtttctaaatataaatgtgaacatacatatttgaaaaatctacctatatgacattaaaatacaattagattttatttgaaataattaaaaactaattggtcacttaataacattaagtgacacataaggaaaatgagttaaataatgtttcttaatgaaataatatttattcttaacattaattaccctaatcatggccttaaacatgctttttgatgatggctgggtcaaagaggtcgccagagttagggaggacagtagtaaggaaacacacctgcaaacatcagaaacattttgatgtatactttcacttatagaaaaagaacaaacaaaaattcgataatttggaaataccctgaacaagtaaaattagcaaacctatagcatattccttattcagggatgggccattgtactatacccctaaacagtccattattatatccctagattactttctatgttaatggaatggaagtctccaacttccattccctagtcttctacctacaagtatataccatccctcttaacaggtctcacagaggagcataagacttaagagccagaaagtaactgataaatcgacaagaagtaagactacctatgaaaggcaggggttgttggagactgccaagaacattaatccatcttcatttccctaatgttcatctttatagtcaatctcacagtatgctatgaaagataagacaatggttaggtttttttaaacatttttaggttaggtaaaatttctgctaatgaatgagaatggtcatcatttaatcaccattatcagaatcaatacaccacccacatcagcatccctagatgtgcaaaggtcttccagtactgcatggctgtgcaaacacagaatctgtgattccgtggttcccttccaccaactgaatcattaggactacagtcctgcaagacaggtgccttgaggcacccaattgtccttcagcatcatgtcctctttctttgtgtcaacatgggagtaagaaggccaggtggtctgaataatgtccataaaattccatcccctattttcccatgtgaccatcttgcttcctggttgctatggattttatctgtgatgtgtagtatctgattcttgctgatccatttgtatacaacaccatgaggaatatgtgcaagtcactgttacatctgggtaatccacaaacctcaaaatgtttctctcttttccaccatggtcaattaaccctccattccagcactctctgcacctccctgaaggtgaaaccagatggctcaagagctgtagttcaggccagttaccttcactattctatcatacagatttctccagagaacattccttctcccaccccagaggaggaaggccccttagcacatgatctctgcggtctccattagtttcaacatcttgtggcgctgatcacttccttttgcctttcaactccatttgatatatgtttcccacgacgtagtggagacttctggctggagaggctggaaaatataactctgaatttcctacaatctcagctccactttctcccgcgcgtaggcccccggctggagcggtgttatt

SEQ ID NO: 18888 - RNA, 1672 nt, Homo sapiens
  source 1..1672: mol_type = other RNA
tgcctactgagctgaaacacagagtggcataaaagaagcacccctgcttattaagcctttaacccaacttcccacaaatggcttcttctgattttctttcagagactgattctgtaatgacttagatgttgtggtttgagaatctgctgtagtttcttttttcttcaaattagatacctgagatgtgacacgttctggttttaattgttcagtttttggtgtaaggaattgttttaactgagcgtccttctcaatttctactgacttcactccctgtataagaccagtagcatcagtattattcacagatttagtatttacagtatcttctgtattcagctgtactgactgcatgtttgtatttacaacttgggatggaaaacttatgtccacaaattggtcttgaataagcttttcattacatggagctgatactgaagaagccattagtgattcttgtgatagcaaagtattggttttgagaattcctgtattttctgctacaggtttattttctaacaggaaagcttcagaatttaactgtgaaactgaggctgttttctggatagtttcttcaagtgtcagaggtaaaatattgtcaaccaaaccttttggacctgaaagtaaatgatctccatgagttacagctgtgtcctgtgaaagagtacgaggggcaactgatatatctttagggtgagttactgaggctgtttcagctgaggcagcatcacccacagaacacgatgttaaagatactggtttctcattactgagagcgtgttggtcattagtctttttaagtggaaggcaggcagcttctttatctgtcacttgggatatttttctttcccaaataacaatatgtatctctgaagcaggaacttcaaatttcttgtgcctttcagaacatgggccttttaagtcatcacattccagccaacttccatcagcatctaaaatccatgttataaaatgattatttgctcgatactgaattacagaagttatctgataaagacagccttcaaaatgaaatgcatagtgctgcaagtcattctgtggtaagccttctacaaagtgcaacatgaatatgggagatactttttctaataccatttttcttatttgtgatttactgttgcaattgttacatggaccaaaatgggcagcattaagtgggtgccactcagggatgacatttgtaaaggtgaccagactcttcatatgcctgttttgatattggtgtccacactgcgaacattcaaagtcccaagaaaaagaatataggaagagcttttcaatgtgggtttctagttttaagagcaggggaaatgcaaacacagggctttccatatcacctaatgtgcatctaagctggggctgaaggctaataaaaatttcatctctaacttcattcagacaggtctctatctctgcaaatatttctgaggtaagttttttacaatctccatctgaactcaaccgtggtctgaaaatattaagcggaaaattccagaaacaatttataagctttaaatttcatgccattctgagtagcatcatgaactctcttgctgtcctgctgtgttccactggcaacgtgaatcttcccttcgtctaatgtgtccatgctgtctacactcctgcctgtggttcacttagcagccatctt

SEQ ID NO: 18889 - RNA, 1738 nt, Homo sapiens
  source 1..1738: mol_type = other RNA
tgcctactgagctgaaacacagagtggcataaaagaagcacccctgcttattaagcctttaacccaacttcccacaaatggcttcttctgattttctttcagagactgattctgtaatgacttagatgttgtggtttgagaatctgctgtagtttcttttttcttcaaattagatacctgagatgtgacacgttctggttttaattgttcagtttttggtgtaaggaattgttttaactgagcgtccttctcaatttctactgacttcactccctgtataagaccagtagcatcagtattattcacagatttagtatttacagtatcttctgtattcagctgtactgactgcatgtttgtatttacaacttgggatggaaaacttatgtccacaaattggtcttgaataagcttttcattacatggagctgatactgaagaagccattagtgattcttgtgatagcaaagtattggttttgagaattcctgtattttctgctacaggtttattttctaacaggaaagcttcagaatttaactgtgaaactgaggctgttttctggatagtttcttcaagtgtcagaggtaaaatattgtcaaccaaaccttttggacctgaaagtaaatgatctccatgagttacagctgtgtcctgtgaaagagtacgaggggcaactgatatatctttagggtgagttactgaggctgtttcagctgaggcagcatcacccacagaacacgatgttaaagatactggtttctcattactgagagcgtgttggtcattagtctttttaagtggaaggcaggcagcttctttatctgtcacttgggatatttttctttcccaaataacaatatgtatctctgaagcaggaacttcaaatttcttgtgcctttcagaacatgggccttttaagtcatcacattccagccaacttccatcagcatctaaaatccatgttataaaatgattatttgctcgatactgaattacagaagttatctgataaagacagccttcaaaatgaaatgcatagtgctgcaagtcattctgtggtaagccttctacaaagtgcaacatgaatatgggagatactttttctaataccatttttcttatttgtgatttactgttgcaattgttacatggaccaaaatgggcagcattaagtgggtgccactcagggatgacatttgtaaaggtgaccagactcttcatatgcctgttttgatattggtgtccacactgcgaacattcaaagtcccaagaaaaagaatataggaagagcttttcaatgtgggtttctagttttaagagcaggggaaatgcaaacacagggctttccatatcacctaatgtgcatctaagctggggctgaaggctaataaaaatttcatctctaacttcattcagacaggtctctatctctgcaaatatttctgaggtaagttttttacaatctccatctgcagatcctcacacaaaaagatagattcttgaaaactaattcggtaagtctttaaggcttttaactttcccttctctctacaagcagggcaatactcatctgatggaactttagctgaatcaaaattctgccgcgggcactccccttcttggtaccgggtcgatcggaactcctgttccagcttgatctccaccctagttgcaacgttcaacccacgttcccctcggactgctcctcccccactcgcgtctccactaggaaggc

SEQ ID NO: 18890 - RNA, 2468 nt, Homo sapiens
  source 1..2468: mol_type = other RNA
tgcctactgagctgaaacacagagtggcataaaagaagcacccctgcttattaagcctttaacccaacttcccacaaatggcttcttctgattttctttcagagactgattctgtaatgacttagatgttgtggtttgagaatctgctgtagtttcttttttcttcaaattagatacctgagatgtgacacgttctggttttaattgttcagtttttggtgtaaggaattgttttaactgagcgtccttctcaatttctactgacttcactccctgtataagaccagtagcatcagtattattcacagatttagtatttacagtatcttctgtattcagctgtactgactgcatgtttgtatttacaacttgggatggaaaacttatgtccacaaattggtcttgaataagcttttcattacatggagctgatactgaagaagccattagtgattcttgtgatagcaaagtattggttttgagaattcctgtattttctgctacaggtttattttctaacaggaaagcttcagaatttaactgtgaaactgaggctgttttctggatagtttcttcaagtgtcagaggtaaaatattgtcaaccaaaccttttggacctgaaagtaaatgatctccatgagttacagctgtgtcctgtgaaagagtacgaggggcaactgatatatctttagggtgagttactgaggctgtttcagctgaggcagcatcacccacagaacacgatgttaaagatactggtttctcattactgagagcgtgttggtcattagtctttttaagtggaaggcaggcagcttctttatctgtcacttgggatatttttctttcccaaataacaatatgtatctctgaagcaggaacttcaaatttcttgtgcctttcagaacatgggccttttaagtcatcacattccagccaacttccatcagcatctaaaatccatgttataaaatgattatttgctcgatactgaattacagaagttatctgataaagacagccttcaaaatgaaatgcatagtgctgcaagtcattctgtggtaagccttctacaaagtgcaacatgaatatgggagatactttttctaataccatttttcttatttgtgatttactgttgcaattgttacatggaccaaaatgggcagcattaagtgggtgccactcagggatgacatttgtaaaggtgaccagactcttcatatgcctgttttgatattggtgtccacactgcgaacattcaaagtcccaagaaaaagaatataggaagagcttttcaatgtgggtttctagttttaagagcaggggaaatgcaaacacagggctttccatatcacctaatgtgcatctaagctggggctgaaggctaataaaaatttcatctctaacttcattcagacaggtctctatctctgcaaatatttctgaggtaagttttttacaatctccatctttaacaccactcaattgactggtatatagaagtgtatttgcttgattatattttgtaagcaaccgccagaatatagattcctccttcgagcacagtccagtcacggtgttctttaactcttccgagtgcaccaaagctgacaggatacagtctaaccaacagagagcataagcatttttccactggacacataaagcctggggaaatgatgtacatttgctctccagtggcatttccagtttagatgtacatccttcattttgaggggaaggtctgccagttccagagacatcaactgtagcaggatcttttgtagtagccatgtcaacagtatcagcttccaaaatctcattccgctccaaggaatcagctgtcctaattggattctgttgaccactactatcaggtaagtttgacgaggtttcgtcatatacttctccattatgtttgctgttcaaaacttttccaccgtcaatagcaatataatttctagtctttttggaatttgctaaaagaagtgaatccttatagctgctttctaagctcttccttttctgaggcttatgtggagtgtgacattcttccaaatcaggagaaattaggttattaagtgatttagagcccaaaggatagatgcactgcagatcctcacacaaaaagatagattcttgaaaactaattcggtaagtctttaaggcttttaactttcccttctctctacaagcagggcaatactcatctgatggaactttagctgaatcaaaattcatgtggagtgaagatatccctatatcagtccctggtccaatcactggcaaaccatttccaatcttcggagaatccatcattccgagtcattggctaatttatgtcacttgagacatgtcaatatcactaaggattttttcaatgaaccctgccgcgggcactccccttcttggtaccgggtcgatcggaactcctgttccagcttgatctccaccctagttgcaac

SEQ ID NO: 18891 - RNA, 2378 nt, Homo sapiens
  source 1..2378: mol_type = other RNA
tgcctactgagctgaaacacagagtggcataaaagaagcacccctgcttattaagcctttaacccaacttcccacaaatggcttcttctgattttctttcagagactgattctgtaatgacttagatgttgtggtttgagaatctgctgtagtttcttttttcttcaaattagatacctgagatgtgacacgttctggttttaattgttcagtttttggtgtaaggaattgttttaactgagcgtccttctcaatttctactgacttcactccctgtataagaccagtagcatcagtattattcacagatttagtatttacagtatcttctgtattcagctgtactgactgcatgtttgtatttacaacttgggatggaaaacttatgtccacaaattggtcttgaataagcttttcattacatggagctgatactgaagaagccattagtgattcttgtgatagcaaagtattggttttgagaattcctgtattttctgctacaggtttattttctaacaggaaagcttcagaatttaactgtgaaactgaggctgttttctggatagtttcttcaagtgtcagaggtaaaatattgtcaaccaaaccttttggacctgaaagtaaatgatctccatgagttacagctgtgtcctgtgaaagagtacgaggggcaactgatatatctttagggtgagttactgaggctgtttcagctgaggcagcatcacccacagaacacgatgttaaagatactggtttctcattactgagagcgtgttggtcattagtctttttaagtggaaggcaggcagcttctttatctgtcacttgggatatttttctttcccaaataacaatatgtatctctgaagcaggaacttcaaatttcttgtgcctttcagaacatgggccttttaagtcatcacattccagccaacttccatcagcatctaaaatccatgttataaaatgattatttgctcgatactgaattacagaagttatctgataaagacagccttcaaaatgaaatgcatagtgctgcaagtcattctgtggtaagccttctacaaagtgcaacatgaatatgggagatactttttctaataccatttttcttatttgtgatttactgttgcaattgttacatggaccaaaatgggcagcattaagtgggtgccactcagggatgacatttgtaaaggtgaccagactcttcatatgcctgttttgatattggtgtccacactgcgaacattcaaagtcccaagaaaaagaatataggaagagcttttcaatgtgggtttctagttttaagagcaggggaaatgcaaacacagggctttccatatcacctaatgtgcatctaagctggggctgaaggctaataaaaatttcatctctaacttcattcagacaggtctctatctctgcaaatatttctgaggtaagttttttacaatctccatctttaacaccactcaattgactggtatatagaagtgtatttgcttgattatattttgtaagcaaccgccagaatatagattcctccttcgagcacagtccagtcacggtgttctttaactcttccgagtgcaccaaagctgacaggatacagtctaaccaacagagagcataagcatttttccactggacacataaagcctggggaaatgatgtacatttgctctccagtggcatttccagtttagatgtacatccttcattttgaggggaaggtctgccagttccagagacatcaactgtagcaggatcttttgtagtagccatgtcaacagtatcagcttccaaaatctcattccgctccaaggaatcagctgtcctaattggattctgttgaccactactatcaggtaagtttgacgaggtttcgtcatatacttctccattatgtttgctgttcaaaacttttccaccgtcaatagcaatataatttctagtctttttggaatttgctaaaagaagtgaatccttatagctgctttctaagctcttccttttctgaggcttatgtggagtgtgacattcttccaaatcaggagaaattaggttattaagtgatttagagcccaaaggatagatgcactgcagatcctcacacaaaaagatagattcttgaaaactaattcggtaagtctttaaggcttttaactttcccttctctctacaagcagggcaatactcatctgatggaactttagctgaatcaaaattctgccgcgggcactccccttcttggtaccgggtcgatcggaactcctgttccagcttgatctccaccctagttgcaacgttcaacccacgttcccctcggactgctcctcccccactcgcgtctccactaggaaggc

SEQ ID NO: 18892 - RNA, 2545 nt, Homo sapiens
  source 1..2545: mol_type = other RNA
tgcctactgagctgaaacacagagtggcataaaagaagcacccctgcttattaagcctttaacccaacttcccacaaatggcttcttctgattttctttcagagactgattctgtaatgacttagatgttgtggtttgagaatctgctgtagtttcttttttcttcaaattagatacctgagatgtgacacgttctggttttaattgttcagtttttggtgtaaggaattgttttaactgagcgtccttctcaatttctactgacttcactccctgtataagaccagtagcatcagtattattcacagatttagtatttacagtatcttctgtattcagctgtactgactgcatgtttgtatttacaacttgggatggaaaacttatgtccacaaattggtcttgaataagcttttcattacatggagctgatactgaagaagccattagtgattcttgtgatagcaaagtattggttttgagaattcctgtattttctgctacaggtttattttctaacaggaaagcttcagaatttaactgtgaaactgaggctgttttctggatagtttcttcaagtgtcagaggtaaaatattgtcaaccaaaccttttggacctgaaagtaaatgatctccatgagttacagctgtgtcctgtgaaagagtacgaggggcaactgatatatctttagggtgagttactgaggctgtttcagctgaggcagcatcacccacagaacacgatgttaaagatactggtttctcattactgagagcgtgttggtcattagtctttttaagtggaaggcaggcagcttctttatctgtcacttgggatatttttctttcccaaataacaatatgtatctctgaagcaggaacttcaaatttcttgtgcctttcagaacatgggccttttaagtcatcacattccagccaacttccatcagcatctaaaatccatgttataaaatgattatttgctcgatactgaattacagaagttatctgataaagacagccttcaaaatgaaatgcatagtgctgcaagtcattctgtggtaagccttctacaaagtgcaacatgaatatgggagatactttttctaataccatttttcttatttgtgatttactgttgcaattgttacatggaccaaaatgggcagcattaagtgggtgccactcagggatgacatttgtaaaggtgaccagactcttcatatgcctgttttgatattggtgtccacactgcgaacattcaaagtcccaagaaaaagaatataggaagagcttttcaatgtgggtttctagttttaagagcaggggaaatgcaaacacagggctttccatatcacctaatgtgcatctaagctggggctgaaggctaataaaaatttcatctctaacttcattcagacaggtctctatctctgcaaatatttctgaggtaagttttttacaatctccatctttaacaccactcaattgactggtatatagaagtgtatttgcttgattatattttgtaagcaaccgccagaatatagattcctccttcgagcacagtccagtcacggtgttctttaactcttccgagtgcaccaaagctgacaggatacagtctaaccaacagagagcataagcatttttccactggacacataaagcctggggaaatgatgtacatttgctctccagtggcatttccagtttagatgtacatccttcattttgaggggaaggtctgccagttccagagacatcaactgtagcaggatcttttgtagtagccatgtcaacagtatcagcttccaaaatctcattccgctccaaggaatcagctgtcctaattggattctgttgaccactactatcaggtaagtttgacgaggtttcgtcatatacttctccattatgtttgctgttcaaaacttttccaccgtcaatagcaatataatttctagtctttttggaatttgctaaaagaagtgaatccttatagctgctttctaagctcttccttttctgaggcttatgtggagtgtgacattcttccaaatcaggagaaattaggttattaagtgatttagagcccaaaggatagatgcactgcagatcctcacacaaaaagatagattcttgaaaactaattcggtaagtctttaaggcttttaactttcccttctctctacaagcagggcaatactcatctgatggaactttagctgaatcaaaattttttcccaaataccccaccatgtggagtgaagatatccctatatcagtccctggtccaatcactggcaaaccatttccaatcttcggagaatccatcattccgagtcattggctaatttatgtcacttgagacatgtcaatatcactaaggattttttcaatgaaccctgccgcgggcactccccttcttggtaccgggtcgatcggaactcctgttccagcttgatctccaccctagttgcaacgttcaacccacgttcccctcggactgctcctcccccactcgcgtctccactaggaaggc

SEQ ID NO: 18893 - RNA, 2325 nt, Homo sapiens
  source 1..2325: mol_type = other RNA
tgcctactgagctgaaacacagagtggcataaaagaagcacccctgcttattaagcctttaacccaacttcccacaaatggcttcttctgattttctttcagagactgattctgtaatgacttagatgttgtggtttgagaatctgctgtagtttcttttttcttcaaattagatacctgagatgtgacacgttctggttttaattgttcagtttttggtgtaaggaattgttttaactgagcgtccttctcaatttctactgacttcactccctgtataagaccagtagcatcagtattattcacagatttagtatttacagtatcttctgtattcagctgtactgactgcatgtttgtatttacaacttgggatggaaaacttatgtccacaaattggtcttgaataagcttttcattacatggagctgatactgaagaagccattagtgattcttgtgatagcaaagtattggttttgagaattcctgtattttctgctacaggtttattttctaacaggaaagcttcagaatttaactgtgaaactgaggctgttttctggatagtttcttcaagtgtcagaggtaaaatattgtcaaccaaaccttttggacctgaaagtaaatgatctccatgagttacagctgtgtcctgtgaaagagtacgaggggcaactgatatatctttagggtgagttactgaggctgtttcagctgaggcagcatcacccacagaacacgatgttaaagatactggtttctcattactgagagcgtgttggtcattagtctttttaagtggaaggcaggcagcttctttatctgtcacttgggatatttttctttcccaaataacaatatgtatctctgaagcaggaacttcaaatttcttgtgcctttcagaacatgggccttttaagtcatcacattccagccaacttccatcagcatctaaaatccatgttataaaatgattatttgctcgatactgaattacagaagttatctgataaagacagccttcaaaatgaaatgcatagtgctgcaagtcattctgtggtaagccttctacaaagtgcaacatgaatatgggagatactttttctaataccatttttcttatttgtgatttactgttgcaattgttacatggaccaaaatgggcagcattaagtgggtgccactcagggatgacatttgtaaaggtgaccagactcttcatatgcctgttttgatattggtgtccacactgcgaacattcaaagtcccaagaaaaagaatataggaagagcttttcaatgtgggtttctagttttaagagcaggggaaatgcaaacacagggctttccatatcacctttaacaccactcaattgactggtatatagaagtgtatttgcttgattatattttgtaagcaaccgccagaatatagattcctccttcgagcacagtccagtcacggtgttctttaactcttccgagtgcaccaaagctgacaggatacagtctaaccaacagagagcataagcatttttccactggacacataaagcctggggaaatgatgtacatttgctctccagtggcatttccagtttagatgtacatccttcattttgaggggaaggtctgccagttccagagacatcaactgtagcaggatcttttgtagtagccatgtcaacagtatcagcttccaaaatctcattccgctccaaggaatcagctgtcctaattggattctgttgaccactactatcaggtaagtttgacgaggtttcgtcatatacttctccattatgtttgctgttcaaaacttttccaccgtcaatagcaatataatttctagtctttttggaatttgctaaaagaagtgaatccttatagctgctttctaagctcttccttttctgaggcttatgtggagtgtgacattcttccaaatcaggagaaattaggttattaagtgatttagagcccaaaggatagatgcactgcagatcctcacacaaaaagatagattcttgaaaactaattcggtaagtctttaaggcttttaactttcccttctctctacaagcagggcaatactcatctgatggaactttagctgaatcaaaattctgccgcgggcactccccttcttggtaccgggtcgatcggaactcctgttccagcttgatctccaccctagttgcaacgttcaacccacgttcccctcggactgctcctcccccactcgcgtctccactaggaaggcggcttccggcttgagtccgcggcaaaagagtcctccttcctgctgcacgctgggcctgaaa

SEQ ID NO: 18894 - RNA, 2463 nt, Homo sapiens
  source 1..2463: mol_type = other RNA
tgcctactgagctgaaacacagagtggcataaaagaagcacccctgcttattaagcctttaacccaacttcccacaaatggcttcttctgattttctttcagagactgattctgtaatgacttagatgttgtggtttgagaatctgctgtagtttcttttttcttcaaattagatacctgagatgtgacacgttctggttttaattgttcagtttttggtgtaaggaattgttttaactgagcgtccttctcaatttctactgacttcactccctgtataagaccagtagcatcagtattattcacagatttagtatttacagtatcttctgtattcagctgtactgactgcatgtttgtatttacaacttgggatggaaaacttatgtccacaaattggtcttgaataagcttttcattacatggagctgatactgaagaagccattagtgattcttgtgatagcaaagtattggttttgagaattcctgtattttctgctacaggtttattttctaacaggaaagcttcagaatttaactgtgaaactgaggctgttttctggatagtttcttcaagtgtcagaggtaaaatattgtcaaccaaaccttttggacctgaaagtaaatgatctccatgagttacagctgtgtcctgtgaaagagtacgaggggcaactgatatatctttagggtgagttactgaggctgtttcagctgaggcagcatcacccacagaacacgatgttaaagatactggtttctcattactgagagcgtgttggtcattagtctttttaagtggaaggcaggcagcttctttatctgtcacttgggatatttttctttcccaaataacaatatgtatctctgaagcaggaacttcaaatttcttgtgcctttcagaacatgggccttttaagtcatcacattccagccaacttccatcagcatctaaaatccatgttataaaatgattatttgctcgatactgaattacagaagttatctgataaagacagccttcaaaatgaaatgcatagtgctgcaagtcattctgtggtaagccttctacaaagtgcaacatgaatatgggagatactttttctaataccatttttcttatttgtgatttactgttgcaattgttacatggaccaaaatgggcagcattaagtgggtgccactcagggatgacatttgtaaaggtgaccagactcttcatatgcctgttttgatattggtgtccacactgcgaacattcaaagtcccaagaaaaagaatataggaagagcttttcaatgtgggtttctagttttaagagcaggggaaatgcaaacacagggctttccatatcacctttaacaccactcaattgactggtatatagaagtgtatttgcttgattatattttgtaagcaaccgccagaatatagattcctccttcgagcacagtccagtcacggtgttctttaactcttccgagtgcaccaaagctgacaggatacagtctaaccaacagagagcataagcatttttccactggacacataaagcctggggaaatgatgtacatttgctctccagtggcatttccagtttagatgtacatccttcattttgaggggaaggtctgccagttccagagacatcaactgtagcaggatcttttgtagtagccatgtcaacagtatcagcttccaaaatctcattccgctccaaggaatcagctgtcctaattggattctgttgaccactactatcaggtaagtttgacgaggtttcgtcatatacttctccattatgtttgctgttcaaaacttttccaccgtcaatagcaatataatttctagtctttttggaatttgctaaaagaagtgaatccttatagctgctttctaagctcttccttttctgaggcttatgtggagtgtgacattcttccaaatcaggagaaattaggttattaagtgatttagagcccaaaggatagatgcactgcagatcctcacacaaaaagatagattcttgaaaactaattcggtaagtctttaaggcttttaactttcccttctctctacaagcagggcaatactcatctgatggaactttagctgaatcaaaattttttcccaaataccccaccatgtggagtgaagatatccctatatcagtccctggtccaatcactggcaaaccatttccaatcttcggagaatccatcattccgagtcattggctaatttatgtcacttgagacatgtcaatatcactaaggattttttcaatgaaccctgccgcgggcactccccttcttggtaccgggtcgatcggaactcctgttccagcttgatctccaccctagttgcaacgttcaacccacgttcccctcggactgctcctcccccactcgcgtctccactaggaaggcggcttccggcttgagtccgcggcaaaagagtc

SEQ ID NO: 18895 - RNA, 3043 nt, Homo sapiens
  source 1..3043: mol_type = other RNA
tgcctactgagctgaaacacaggagggtttgggttgacaggtgagaaaactgttagcaaacacctggtgaagagcaggagtgggagcgggaggagacagactgaggagggccccagggcttgctgttgcccagaaagccacccggccctgccatacgctgccagcagtgcagggtaaccaaggcaggacctgggcgtgggggacctcagggcaggccggggcctcctttgaggcagagcttgccgtcagcctgagagtcccatttgttgacgttctcacatccggagcactggctaatctgtaaccacaggtcagcctgcagccgcctggcttgctagcaggtatctgctggcccctgtttgggaggcgctgccagccctttactgtctccacaaacatcctcctgctggtccgcatctggcacggggcatgggagggagccgggaagtgcgggtgcctggcttagacaggcaagggggttctccacccctcccagcacccacctccaccctctccctttaaacccaaccatgggaaatttaggagaaacaaacatgctttctggggctcacagagggaagggcagaacatcctaaaatcactcacagtcacagactttaagattcagagaatcttcaagccacgggatctcatagatttatagaatcatctggtctagtgggtctcaaacttttttaaaaagcagtggaatccttttgtccaacagaaccccaagttctggctgaagtctaggaggtggacctagcacctatcccctcaccctctctctggccttctctgcagcctccaagacacctctgtggaaccccagtgttccaaggaacccagctggagaagcacagatcttgttccaaggagcaatttcgattgcatggttttcctttcagcccgatacagagacctgggttcaaggctccctcttctagttgaagagctggtttgaggggttggcttttttggccgtggagggcggtgtctttaaattaggtattcctttttaacctaaagacaaaagcccttctcatttgtgtaaatgcctttccacatctgtgaggtaagtggggtgtgtataattatgcccaaataatgaggaggctgaagcacagagaagctgagaactgcccagagctaatgagtggccaagtcaagccttgattcagtgggtctcctgcatcttaaatgaaggcattgtccccaatactgcaaggcccgagctcctccctccacatacaccccaccctgagccccaccactctctccaaggccccagtacaatctcttgggcccaagagatgctaggggcaaacatgagattgcctttcttgtaagttaaaaacagtccaatactggtgattacatatggttcaacttgatatatattcattgtggtagaaaactagagtgcacaggaataactgaaccagacaaagccctcgggagcctccggggaactataaggcaggcagaccgaccttccccactgaatctggcatcctgggcgctgcactgcccctcttccttgtaccagcactgctggggccctggtggcctatctgtgcccaacatgtgcagttgatccttgatgccttgagctcttgtaagctcgactctggaaggcacaggagggccactgtccccgctcttgtcgggtatccagaccaagcagctggacgccccgcgtgaggccgtagacgtccaccagggcccagagcgggtcggccgtgcggaccccgctgaagaacagcataacagccgagtcgttgatgcggtggaagacacggcccttcttgtccacccagaatgcgatgatgttgccctcattggcaaactcctcaggcagcgccttggcccagaagccactctgggacaccaggtcggggcaggcgtacttgggcagcgagtcagggtggatgcgggacgggtccttgctggtgaagcccagccgcagggccccgctccagcagcactgcttcttggtgatcttcagcctgacttgctcgtagatgaggaccgggcggttgctgaaggtgatggcgttgcagaagctggcctgcctcttgacagccttgtggctgaggtccatgaggatctgggagcccttggtgtgcgggtggaagagcagcggcgtggctgggagccccccgctgggcagcactgccggacagtgcttctgcttgtggtggcatcggtgagaagtgacggggaaggggcccccgatagagtcccaaattttttcttgcataagatccaagaaccctctcttggggtctgaattgtgaccgctttccagtaacatcttccatggtgaatcacaaagggatgatactgaagagacccctttgaggttctgggggtggccccgcggcgcgcggctcgggtttcctcggggcagcgaggggatactggagaagttgttacccatggcatccggccccaggaggttcggcgctcgcgggtgggggcgaggccgggcaggcgctgaggtgcggtgtgcgagtgtgcgcgcgcgggtgcgcgccaccgggggagggccctgctggggctgcagccgggggcgggcgggcagctcctcagcttcctttctctggacttcgcggtccttggcgggttccgcccgccacgggtgtcctggcgcaggctgggctacctgcctcccatgccccgtggcgggagcgggggccacaagcagggccctgggccggggccggggacgcccggggctccccgcttgctccccgggacgctagggttccggctgggggtgggcggcgcggcggctccggcgcgctcccccggggccatagagtcagggtcgctggcgtgggcgttcggcggctccgaggcaggctcggttaccgccccgcggagacggccgcggcggcgatgtgcgtggctccctcccgcccgcgggtctgcgtggagcggggctcggcggagcgcggggcgttctgggcgctccgacgcagctggtgtcccccgaccgccgcggtcccgcccgcgccgggtccctcctgcgaccgcc

SEQ ID NO: 18896 - RNA, 3576 nt, Homo sapiens
  source 1..3576: mol_type = other RNA
tgcctactgagctgaaacacagggcttcgcaacgactcactctctttggcacagggatgactcaggacaataaagagaagccccatttcagaataggctttgtgacagactgaagcttggtaagaatcatcaatgtgcatctttttcaggagttgaccagtttttaaattccaaataacaatgttgttcataatagtagtaccaagcagagcttcttgcatcccttggacctcagcaaaagttagtatagtctcctcagggggcatcaaaaattggttttctttgcctcctccatcttctgcaaacgtcatgacttctacttgttgatcagaaagggtcccactgctactaactagcctcctctttgtcaggccaagcacagcttttatatttccagacttcagtagtacttgcttttcactttcatcatcagaggaacaaaacaatgccctgatctctctgatttccaaatttcccaaagctacacacacgagattatacacatcaggcactggaactatctgtaatactggaacctctgcgaagtgccaggtataaagtttttcccactgccaagcatccagagctttccaaagagaaactacatcttcgcaagcagttatgatacatggctctttacaaccggctctttcccaaaacatggcactcacatctacggaacaggaacctgaaggattctttaactctgaaaccaattgtaggttgcctgggtttatgctatcagaagcaggaagctctgctgtttcagtctgttcgacggaatgtttatgcagctcctggcatgtgtttctacagagctgattttctttaaaagtgaatgactcaatgggtggaggtgttcctggcgggacagagtcacagtcacaggtaggttgtccttgcctgcctgacacttgcagggtggtatgtggttttgctgggctgcctgaactgtcgaattgtttagtatcactggcaagacagactgagtctttcaaatgagcaagttggggtgtgcagcaagttcgtccagcaacttctgtagatgctttttcataggagccttgagggccaaaggctggagtagtacctaagatggggaaagcaggtgaacacatgtctgtggtaggcctgtcattatcatcaggcgcaaccgtatttaaaggagtataaagtaatatggatgaagaaaggcccgtctttgtatgctggctttgcgagtttggccttttgggatgtgattttcctggtagaacaataaggtcctcttctaagtcctccatttctgtatccatgcgtttaggactcagttcctctggaaaaatacagcttccctctttaagatgtctctctccaaacatttttgactcaaagggctccactggtttttctgagcaggacttcactttttcaagcttaagaggtccaaagtcttcatcaggtaactgaaagtctgtgatactgagaaaagacagtagttgctttaaactcagcattccatccctatgaaatggagccgtgaaagcatcatcatccaaggataaataagcactattactccaagaaagggaatcctctttttgatgacgacttttcttccctttcacttgaataaataatttttcgtgctgatatttgtgtgaggtgacttcttccttggacctgttaacaatcgacaggctagaagttggcaaaagtggttcacaatgatctgatgctggggtgcaggctgattttctttttcctgtgtatcttctaccaggtgcttgggcaactgccttcctagacaagtcattatcttcagtgggcccagcgggagagctgactttagttaatgagagaagtttctgagaggttcttgaacttggttgtcctgtgcatgtgccagacatcctaatttcactttggtcagtttcctcattggaaaggtttaaatttttacttgcatccttatttttatttttaaacccttttttcttgacatccaaatgactctgaatgacagcctccacggctactttcctctggcaattggacatgcttcgtgttgttctaacataatattctgcaggaaacagaaggccttcaggcactgtgcaagaatgtttttctgcagaaagaggagaggttgcttccaggctaagactcttaggttgacttagaatctcactttcctgaagattttcattcctgccatcaagagtgtcactgggagattttaaagatttctctgtttgattttgttcttttaagttttggttttcatttgctggtaagttattgtaggtgagttcatttagagaacatgaaatatttgcctctaaattagaacttgtgggcagttggccacttttacttatagctttatttacaaggaggttatctgtagagacagtcatttttttgccttgtgcctccaaacttacaggtgaagtaaatctaatgttttttaggtcgtgagtagtaagttcactgctacctttaggaggaatgtgttcaaggtgctgactactaccgctatctgatagagtctgtaaaggaactgtagtcgccctggtgaaattaggtcttcttaggaatgtatcaacacctttttctggttgggcagttggtggaattaatacactgtcttcattaatttctgtaactggttctggagaatctggaagttcagatttaagacttaaaaggtgagttcttatttcagttactggtgatctagcaggatttttgctactgatttcttcctgttcctttagtcttttcccagacaatctgagtgaatcagtgccaaagacacagtctctctcctgtgaaataaatgtcctcttctgctgcttctttcttctgcttggcagcttctgcttttgctcaccactagggtcactgaccctgtggggaaaatgttcttgggtgtcatctgttctttgtataggtaatcctcctgggccatctccagggttaaaggactcaggcccaacatcaagtgtgatagatgtcttttctccagtttcttcatcaagatgggttttgatgtgtaacttgtcataaacacatattttatttttaggttctgagtgttttagctgcggtgagagatcctgctgagacaaacaatcttgttcttctactgttttcttaatagaatgcttaatcttttcagctctttgggcacgctgaaggcgggctagtgtcttgctgtattcccttttcaagaatgctaatttctcctttaacacagtattctcacactatgttctctgtttctccccatcatccagatccttgaaggtagcaggaactgccatcctcagtcactcaacaaatgaatcttctatttatccgttaatggtccaggtatctctagtaccttttccttctcctcacagctgaggggcttcccgggaggctcgtccatcgggcaggcgacagaacgaaaagagcagccgtcgccgaccccaggcctgccgacaccgggacccagttggccctgggccggggaggcgccccaggaaggaatggggagcccgggatcgcaccctcagtgcgcgatcagctgacccacgcgggccaagc

SEQ ID NO: 18897 - RNA, 4289 nt, Homo sapiens
  source 1..4289: mol_type = other RNA
tgcctactgagctgaaacacagggcttcgcaacgactcactctctttggcacagggatgactcaggacaataaagagaagccccatttcagaataggctttgtgacagactgaagcttggtaagaatcatcaatgtgcatctttttcaggagttgaccagtttttaaattccaaataacaatgttgttcataatagtagtaccaagcagagcttcttgcatcccttggacctcagcaaaagttagtatagtctcctcagggggcatcaaaaattggttttctttgcctcctccatcttctgcaaacgtcatgacttctacttgttgatcagaaagggtcccactgctactaactagcctcctctttgtcaggccaagcacagcttttatatttccagacttcagtagtacttgcttttcactttcatcatcagaggaacaaaacaatgccctgatctctctgatttccaaatttcccaaagctacacacacgagattatacacatcaggcactggaactatctgtaatactggaacctctgcgaagtgccaggtataaagtttttcccactgccaagcatccagagctttccaaagagaaactacatcttcgcaagcagttatgatacatggctctttacaaccggctctttcccaaaacatggcactcacatctacggaacaggaacctgaaggattctttaactctgaaaccaattgtaggttgcctgggtttatgctatcagaagcaggaagctctgctgtttcagtctgttcgacggaatgtttatgcagctcctggcatgtgtttctacagagctgattttctttaaaagtgaatgactcaatgggtggaggtgttcctggcgggacagagtcacagtcacaggtaggttgtccttgcctgcctgacacttgcagggtggtatgtggttttgctgggctgcctgaactgtcgaattgtttagtatcactggcaagacagactgagtctttcaaatgagcaagttggggtgtgcagcaagttcgtccagcaacttctgtagatgctttttcataggagccttgagggccaaaggctggagtagtacctaagatggggaaagcaggtgaacacatgtctgtggtaggcctgtcattatcatcaggcgcaaccgtatttaaaggagtataaagtaatatggatgaagaaaggcccgtctttgtatgctggctttgcgagtttggccttttgggatgtgattttcctggtagaacaataaggtcctcttctaagtcctccatttctgtatccatgcgtttaggactcagttcctctggaaaaatacagcttccctctttaagatgtctctctccaaacatttttgactcaaagggctccactggtttttctgagcaggacttcactttttcaagcttaagaggtccaaagtcttcatcaggtaactgaaagtctgtgatactgagaaaagacagtagttgctttaaactcagcattccatccctatgaaatggagccgtgaaagcatcatcatccaaggataaataagcactattactccaagaaagggaatcctctttttgatgacgacttttcttccctttcacttgaataaataatttttcgtgctgatatttgtgtgaggtgacttcttccttggacctgttaacaatcgacaggctagaagttggcaaaagtggttcacaatgatctgatgctggggtgcaggctgattttctttttcctgtgtatcttctaccaggtgcttgggcaactgccttcctagacaagtcattatcttcagtgggcccagcgggagagctgactttagttaatgagagaagtttctgagaggttcttgaacttggttgtcctgtgcatgtgccagacatcctaatttcactttggtcagtttcctcattggaaaggtttaaatttttacttgcatccttatttttatttttaaacccttttttcttgacatccaaatgactctgaatgacagcctccacggctactttcctctggcaattggacatgcttcgtgttgttctaacataatattctgcaggaaacagaaggccttcaggcactgtgcaagaatgtttttctgcagaaagaggagaggttgcttccaggctaagactcttaggttgacttagaatctcactttcctgaagattttcattcctgccatcaagagtgtcactgggagattttaaagatttctctgtttgattttgttcttttaagttttggttttcatttgctggtaagttattgtaggtgagttcatttagagaacatgaaatatttgcctctaaattagaacttgtgggcagttggccacttttacttatagctttatttacaaggaggttatctgtagagacagtcatttttttgccttgtgcctccaaacttacaggtgaagtaaatctaatgttttttaggtcgtgagtagtaagttcactgctacctttaggaggaatgtgttcaaggtgctgactactaccgctatctgatagagtctgtaaaggaactgtagtcgccctggtgaaattaggtcttcttaggaatgtatcaacacctttttctggttgggcagttggtggaattaatacactgtcttcattaatttctgtaactggttctggagaatctggaagttcagatttaagacttaaaaggtgagttcttatttcagttactggtgatctagcaggatttttgctactgatttcttcctgttcctttagtcttttcccagacaatctgagtgaatcagtgccaaagacacagtctctctcctgtgaaataaatgtcctcttctgctgcttctttcttctgcttggcagcttctgcttttgctcaccactagggtcactgaccctgtggggaaaatgttcttgggtgtcatctgttctttgtataggtaatcctcctgggccatctccagggttaaaggactcaggcccaacatcaagtgtgatagatgtcttttctccagtttcttcatcaagatgggttttgatgtgtaacttgtcataaacacatattttatttttaggttctgagtgttttagctgcggtgagagatcctgctgagacaaacaatcttgttcttctactgttttcttaatagaatgcttaatcttttcagctctttgggcacgctgaaggcgggctagtgtcttgctgtattcccttttcaagaatgctaatttctcctttaactccaccagaaggtaagccaggataagaataacatcagcacaagctggaaacatcctaaaagtctatcagtaaagtacagtctaaagaagcaagggcacttccaaggccaggtgcagtggcgggttcgtgtaatcccagctactcgggaggctgaggcaggagagtcgcttgatcccaggaagcggaggttgcagtgagccgagatcgcgccactgcaccccagcatgggtggcagagtgagactctgtctcaaaaaagaagaaaaacagaaaaggaagaaaaaagaaacaaaacgagggcacttccaaactacaacatactgtctagaacttaaaaaagaaagcaaggtagataaacatgtcctgacaggaaagctaaacggaacctgcagaaccattcagatcataccatttatgaacattcccttctccaaaaaatatacataggattcctttttggtggttagggatacgcccctcctccaccacccacattaacacacgaaaggacctggaagtaccagacttaaaagatttacttgaggccgtccggggggagaagtaaagattgagggtgtgggaggggggaggagcaagggtgtcgatacagctttatctacaaactgttacacattgtattaatgcgctgctactgtaatgaaatttgttctttaaacgccaccacgtgagcaccacgctatttccacattttcattttctgtgccccctcagccctaagaggagggggtggtcagatgatactgctgccctcggactgccgaggacacaaagccaggcctaaaaccctgggaaagcggggtcagagtcctgcgtccgcccttcccgcacccccggcaccttttccttctcctcacagctgaggggcttcccgggaggctcgtccatcgggcaggcgacagaacgaaaagagcagccgtcgccgaccccaggcctgccgacaccgggacccagttggccctgggccggggaggcgccccaggaaggaatggggagcccgggatcgcaccctcagtgcgcgatcagctgacccac

SEQ ID NO: 18898 - RNA, 3437 nt, Homo sapiens
  source 1..3437: mol_type = other RNA
tgcctactgagctgaaacacagggcttcgcaacgactcactctctttggcacagggatgactcaggacaataaagagaagccccatttcagaataggctttgtgacagactgaagcttggtaagaatcatcaatgtgcatctttttcaggagttgaccagtttttaaattccaaataacaatgttgttcataatagtagtaccaagcagagcttcttgcatcccttggacctcagcaaaagttagtatagtctcctcagggggcatcaaaaattggttttctttgcctcctccatcttctgcaaacgtcatgacttctacttgttgatcagaaagggtcccactgctactaactagcctcctctttgtcaggccaagcacagcttttatatttccagacttcagtagtacttgcttttcactttcatcatcagaggaacaaaacaatgccctgatctctctgatttccaaatttcccaaagctacacacacgagattatacacatcaggcactggaactatctgtaatactggaacctctgcgaagtgccaggtataaagtttttcccactgccaagcatccagagctttccaaagagaaactacatcttcgcaagcagttatgatacatggctctttacaaccggctctttcccaaaacatggcactcacatctacggaacaggaacctgaaggattctttaactctgaaaccaattgtaggttgcctgggtttatgctatcagaagcaggaagctctgctgtttcagtctgttcgacggaatgtttatgcagctcctggcatgtgtttctacagagctgattttctttaaaagtgaatgactcaatgggtggaggtgttcctggcgggacagagtcacagtcacaggtaggttgtccttgcctgcctgacacttgcagggtggtatgtggttttgctgggctgcctgaactgtcgaattgtttagtatcactggcaagacagactgagtctttcaaatgagcaagttggggtgtgcagcaagttcgtccagcaacttctgtagatgctttttcataggagccttgagggccaaaggctggagtagtacctaagatggggaaagcaggtgaacacatgtctgtggtaggcctgtcattatcatcaggcgcaaccgtatttaaaggagtataaagtaatatggatgaagaaaggcccgtctttgtatgctggctttgcgagtttggccttttgggatgtgattttcctggtagaacaataaggtcctcttctaagtcctccatttctgtatccatgcgtttaggactcagttcctctggaaaaatacagcttccctctttaagatgtctctctccaaacatttttgactcaaagggctccactggtttttctgagcaggacttcactttttcaagcttaagaggtccaaagtcttcatcaggtaactgaaagtctgtgatactgagaaaagacagtagttgctttaaactcagcattccatccctatgaaatggagccgtgaaagcatcatcatccaaggataaataagcactattactccaagaaagggaatcctctttttgatgacgacttttcttccctttcacttgaataaataatttttcgtgctgatatttgtgtgaggtgacttcttccttggacctgttaacaatcgacaggctagaagttggcaaaagtggttcacaatgatctgatgctggggtgcaggctgattttctttttcctgtgtatcttctaccaggtgcttgggcaactgccttcctagacaagtcattatcttcagtgggcccagcgggagagctgactttagttaatgagagaagtttctgagaggttcttgaacttggttgtcctgtgcatgtgccagacatcctaatttcactttggtcagtttcctcattggaaaggtttaaatttttacttgcatccttatttttatttttaaacccttttttcttgacatccaaatgactctgaatgacagcctccacggctactttcctctggcaattggacatgcttcgtgttgttctaacataatattctgcaggaaacagaaggccttcaggcactgtgcaagaatgtttttctgcagaaagaggagaggttgcttccaggctaagactcttaggttgacttagaatctcactttcctgaagattttcattcctgccatcaagagtgtcactgggagattttaaagatttctctgtttgattttgttcttttaagttttggttttcatttgctggtaagttattgtaggtgagttcatttagagaacatgaaatatttgcctctaaattagaacttgtgggcagttggccacttttacttatagctttatttacaaggaggttatctgtagagacagtcatttttttgccttgtgcctccaaacttacaggtgaagtaaatctaatgttttttaggtcgtgagtagtaagttcactgctacctttaggaggaatgtgttcaaggtgctgactactaccgctatctgatagagtctgtaaaggaactgtagtcgccctggtgaaattaggtcttcttaggaatgtatcaacacctttttctggttgggcagttggtggaattaatacactgtcttcattaatttctgtaactggttctggagaatctggaagttcagatttaagacttaaaaggtgagttcttatttcagttactggtgatctagcaggatttttgctactgatttcttcctgttcctttagtcttttcccagacaatctgagtgaatcagtgccaaagacacagtctctctcctgtgaaataaatgtcctcttctgctgcttctttcttctgcttggcagcttctgcttttgctcaccactagggtcactgaccctgtggggaaaatgttcttgggtgtcatctgttctttgtataggtaatcctcctgggccatctccagggttaaaggactcaggcccaacatcaagtgtgatagatgtcttttctccagtttcttcatcaagatgggttttgatgtgtaacttgtcataaacacatattttatttttaggttctgagtgttttagctgcggtgagagatcctgctgagacaaacaatcttgttcttctactgttttcttaatagaatgcttaatcttttcagctctttgggcacgctgaaggcgggctagtgtcttgctgtattcccttttcaagaatgctaatttctcctttaacttttccttctcctcacagctgaggggcttcccgggaggctcgtccatcgggcaggcgacagaacgaaaagagcagccgtcgccgaccccaggcctgccgacaccgggacccagttggccctgggccggggaggcgccccaggaaggaatggggagcccgggatcgcaccctcagtgcgcgatcagctgacccacgcgggc

SEQ ID NO: 18899 - RNA, 1574 nt, Homo sapiens
  source 1..1574: mol_type = other RNA
tgcctactgagctgaaacacagtctagaacaggagatggttcaggttctccggaggctggcatactctcaagacttgtgtccagttcgttattggtgttttctttacactgctcttttgaggcactgctatctcccaccacatctacttcctcctcagaatcccttaaagatgactgagtttcagaaaagggccctgtagctggctcagtagtcagctgattaacatgttccacaggcaagcaggcagttactattttgtggtcctccaacttgacctgcacttgtgaatctgtgcaaggcaccttatggtctatataactgtcctccttcctactatcaaggaacattgaagtttgggtatccgtatccccattttcagctactgatttttcctgtaacacataggaaccaatgctattttgtttagtgttcccatcaggctgacagtcatcacagtttataacagctgaatcactgtcatcaacaccattgacagccaaatagcctgtgatttcttcaactactgcagaattaagtggcccttcctcactgacattcacctttttaatttcccttttctcacaatcatccagtataagacatcgacaagctcgtttagtcccttgaaaatctgcatcattgtccactactgtactcctctgttctactgactccttgtctgattttataggagaatcttcttctgaactgtttggtgcttcagatctaagacaacgcttaattctttttaaaactggtgaaacaggttctgtttgccttctctcacaattttctatagcctgcctttctatgttatccttttctgaagaagaaagtcctcttttcctagggcttacccatgattctcgggtactctgctgttttaaatcagtggttctcccattattatttcctttctgaattggcacaggctctggtctcttctttggtgatcttgatcgtacttgagaattagaagagatttcttcaggatgcgcaatgctacgattccttaaagttctaccacaaaaagattcatccaagccgtttaaccccactgttgatcttgtaacacgagtagatcgggaagcagccatactatggcaagtccctacaatacggtcatcatgatccactcattgggaaacctgtacaaccaaagatctatcattgtggaaatataatctcttttccttatatcctgaaggagttggagctatgatctagaatggagcttaagcatcagggtttcagactctctcagcttcagccatgaagaatactagaacctcctaaatttttagctgagctctatcagcattaagatagacaggatcctgcagtgtttcttaaaagcctgatacacttttaaaaagcgttttgcctagtatttgatccccatgcgtctgtatttatctgtcatcactgttaattgtccatgttacactgagacttcaggtattatttatttatatggttgtactagaataacttgatatcttgtagaaagagttgcaggtcccaggcccccggaacccaaggctccgccatccaggacaactgctctgccaac

SEQ ID NO: 18900 - RNA, 1637 nt, Homo sapiens
  source 1..1637: mol_type = other RNA
tgcctactgagctgaaacacagtctagaacaggagatggttcaggttctccggaggctggcatactctcaagacttgtgtccagttcgttattggtgttttctttacactgctcttttgaggcactgctatctcccaccacatctacttcctcctcagaatcccttaaagatgactgagtttcagaaaagggccctgtagctggctcagtagtcagctgattaacatgttccacaggcaagcaggcagttactattttgtggtcctccaacttgacctgcacttgtgaatctgtgcaaggcaccttatggtctatataactgtcctccttcctactatcaaggaacattgaagtttgggtatccgtatccccattttcagctactgatttttcctgtaacacataggaaccaatgctattttgtttagtgttcccatcaggctgacagtcatcacagtttataacagctgaatcactgtcatcaacaccattgacagccaaatagcctgtgatttcttcaactactgcagaattaagtggcccttcctcactgacattcacctttttaatttcccttttctcacaatcatccagtataagacatcgacaagctcgtttagtcccttgaaaatctgcatcattgtccactactgtactcctctgttctactgactccttgtctgattttataggagaatcttcttctgaactgtttggtgcttcagatctaagacaacgcttaattctttttaaaactggtgaaacaggttctgtttgccttctctcacaattttctatagcctgcctttctatgttatccttttctgaagaagaaagtcctcttttcctagggcttacccatgattctcgggtactctgctgttttaaatcagtggttctcccattattatttcctttctgaattggcacaggctctggtctcttctttggtgatcttgatcgtacttgagaattagaagagatttcttcaggatgcgcaatgctacgattccttaaagttctaccacaaaaagattcatccaagccgtttaaccccactgttgatcttgtaacacgagtagatcgggaagcagccatactatggcaagtccctacaatacggtcatcatgatccactcattgggaaacctgtacaaccaaagatctatcattgtggaaatataatctcttttccttatatcctgaaggagttggagctatgatctagaatggagcttaagcatcagggtttcagactctctcagcttcagccatgaagaatactagaacctcctaaatttttagctgagctctatcagcattaagatagacaggatcctgcagtgtttcttaaaagcctgatacacttttaaaaagcgttttgcctagtatttgatccccatgcgtctgtatttatctgtcatcactgttaattgtccatgttacactgagacttcaggtattatttatttatatggttgtactagaataacttgatatctttcacgcggggtcggacgcaacgggccacttggggaggcgccgccgccgtggccgctctccgcccccgccacggcacttgctcgggtggccaccgctgcaggaagctcgatagcggcgccgcggcgcttccaggt

SEQ ID NO: 18901 - RNA, 1649 nt, Homo sapiens
  source 1..1649: mol_type = other RNA
tgcctactgagctgaaacacagtctagaacaggagatggttcaggttctccggaggctggcatactctcaagacttgtgtccagttcgttattggtgttttctttacactgctcttttgaggcactgctatctcccaccacatctacttcctcctcagaatcccttaaagatgactgagtttcagaaaagggccctgtagctggctcagtagtcagctgattaacatgttccacaggcaagcaggcagttactattttgtggtcctccaacttgacctgcacttgtgaatctgtgcaaggcaccttatggtctatataactgtcctccttcctactatcaaggaacattgaagtttgggtatccgtatccccattttcagctactgatttttcctgtaacacataggaaccaatgctattttgtttagtgttcccatcaggctgacagtcatcacagtttataacagctgaatcactgtcatcaacaccattgacagccaaatagcctgtgatttcttcaactactgcagaattaagtggcccttcctcactgacattcacctttttaatttcccttttctcacaatcatccagtataagacatcgacaagctcgtttagtcccttgaaaatctgcatcattgtccactactgtactcctctgttctactgactccttgtctgattttataggagaatcttcttctgaactgtttggtgcttcagatctaagacaacgcttaattctttttaaaactggtgaaacaggttctgtttgccttctctcacaattttctatagcctgcctttctatgttatccttttctgaagaagaaagtcctcttttcctagggcttacccatgattctcgggtactctgctgttttaaatcagtggttctcccattattatttcctttctgaattggcacaggctctggtctcttctttggtgatcttgatcgtacttgagaattagaagagatttcttcaggatgcgcaatgctacgattccttaaagttctaccacaaaaagattcatccaagccgtttaaccccactgttgatcttgtaacacgagtagatcgggaagcagccatactatggcaagtccctacaatacggtcatcatgatccactcattgggaaacctgtacaaccaaagatctatcattgtggaaatataatctcttttccttatatcctgaaggagttggagctatgatctagaatggagcttaagcatcagggtttcagactctctcagcttcagccatgaagaatactagaacctcctaaatttttagctgagctctatcagcattaagatagacaggatcctgcagtgtttcttaaaagcctgatacacttttaaaaagcgttttgcctagtatttgatccccatgcgtctgtatttatctgtcatcactgttaattgtccatgttacactgagacttcaggtattatttatttatatggttgtactagaataacttgatatctttcacgcggggtcggacgcaacgggccacttggggaggcgccgccgccgtggccgctctccgcccccgccacggcacttgctcgggtggccaccgctgcaggaagctcgatagcggcgccgcggcgcttccaggtgggtccccgcct

SEQ ID NO: 18902 - RNA, 1511 nt, Homo sapiens
  source 1..1511: mol_type = other RNA
tgcctactgagctgaaacacagtctagaacaggagatggttcaggttctccggaggctggcatactctcaagacttgtgtccagttcgttattggtgttttctttacactgctcttttgaggcactgctatctcccaccacatctacttcctcctcagaatcccttaaagatgactgagtttcagaaaagggccctgtagctggctcagtagtcagctgattaacatgttccacaggcaagcaggcagttactattttgtggtcctccaacttgacctgcacttgtgaatctgtgcaaggcaccttatggtctatataactgtcctccttcctactatcaaggaacattgaagtttgggtatccgtatccccattttcagctactgatttttcctgtaacacataggaaccaatgctattttgtttagtgttcccatcaggctgacagtcatcacagtttataacagctgaatcactgtcatcaacaccattgacagccaaatagcctgtgatttcttcaactactgcagaattaagtggcccttcctcactgacattcacctttttaatttcccttttctcacaatcatccagtataagacatcgacaagctcgtttagtcccttgaaaatctgcatcattgtccactactgtactcctctgttctactgactccttgtctgattttataggagaatcttcttctgaactgtttggtgcttcagatctaagacaacgcttaattctttttaaaactggtgaaacaggttctgtttgccttctctcacaattttctatagcctgcctttctatgttatccttttctgaagaagaaagtcctcttttcctagggcttacccatgattctcgggtactctgctgttttaaatcagtggttctcccattattatttcctttctgaattggcacaggctctggtctcttctttggtgatcttgatcgtacttgagaattagaagagatttcttcaggatgcgcaatgctacgattccttaaagttctaccacaaaaagattcatccaagccgtttaaccccactgttgatcttgtaacacgagtagatcgggaagcagccatactatggcaagtccctacaatacggtcatcatgatccactcattgggaaacctgtacaaccaaagatctatcattgtggaaatataatctcttttccttatatcctgaaggagttggagctatgatctagaatggagcttaagcatcagggtttcagactctctcagcttcagccatgaagaatactagaacctcctaaatttttcttttaaaaagcgttttgcctagtatttgatccccatgcgtctgtatttatctgtcatcactgttaattgtccatgttacactgagacttcaggtattatttatttatatggttgtactagaataacttgatatcttgtagaaagagttgcaggtcccaggcccccggaacccaaggctccgccatccaggacaactgctctgccaac

SEQ ID NO: 18903 - RNA, 1574 nt, Homo sapiens
  source 1..1574: mol_type = other RNA
tgcctactgagctgaaacacagtctagaacaggagatggttcaggttctccggaggctggcatactctcaagacttgtgtccagttcgttattggtgttttctttacactgctcttttgaggcactgctatctcccaccacatctacttcctcctcagaatcccttaaagatgactgagtttcagaaaagggccctgtagctggctcagtagtcagctgattaacatgttccacaggcaagcaggcagttactattttgtggtcctccaacttgacctgcacttgtgaatctgtgcaaggcaccttatggtctatataactgtcctccttcctactatcaaggaacattgaagtttgggtatccgtatccccattttcagctactgatttttcctgtaacacataggaaccaatgctattttgtttagtgttcccatcaggctgacagtcatcacagtttataacagctgaatcactgtcatcaacaccattgacagccaaatagcctgtgatttcttcaactactgcagaattaagtggcccttcctcactgacattcacctttttaatttcccttttctcacaatcatccagtataagacatcgacaagctcgtttagtcccttgaaaatctgcatcattgtccactactgtactcctctgttctactgactccttgtctgattttataggagaatcttcttctgaactgtttggtgcttcagatctaagacaacgcttaattctttttaaaactggtgaaacaggttctgtttgccttctctcacaattttctatagcctgcctttctatgttatccttttctgaagaagaaagtcctcttttcctagggcttacccatgattctcgggtactctgctgttttaaatcagtggttctcccattattatttcctttctgaattggcacaggctctggtctcttctttggtgatcttgatcgtacttgagaattagaagagatttcttcaggatgcgcaatgctacgattccttaaagttctaccacaaaaagattcatccaagccgtttaaccccactgttgatcttgtaacacgagtagatcgggaagcagccatactatggcaagtccctacaatacggtcatcatgatccactcattgggaaacctgtacaaccaaagatctatcattgtggaaatataatctcttttccttatatcctgaaggagttggagctatgatctagaatggagcttaagcatcagggtttcagactctctcagcttcagccatgaagaatactagaacctcctaaatttttcttttaaaaagcgttttgcctagtatttgatccccatgcgtctgtatttatctgtcatcactgttaattgtccatgttacactgagacttcaggtattatttatttatatggttgtactagaataacttgatatctttcacgcggggtcggacgcaacgggccacttggggaggcgccgccgccgtggccgctctccgcccccgccacggcacttgctcgggtggccaccgctgcaggaagctcgatagcggcgccgcggcgcttccaggt

SEQ ID NO: 18904 - RNA, 1420 nt, Homo sapiens
  source 1..1420: mol_type = other RNA
tgcctactgagctgaaacacagtctagaacaggagatggttcaggttctccggaggctggcatactctcaagacttgtgtccagttcgttattggtgttttctttacactgctcttttgaggcactgctatctcccaccacatctacttcctcctcagaatcccttaaagatgactgagtttcagaaaagggccctgtagctggctcagtagtcagctgattaacatgttccacaggcaagcaggcagttactattttgtggtcctccaacttgacctgcacttgtgaatctgtgcaaggcaccttatggtctatataactgtcctccttcctactatcaaggaacattgaagtttgggtatccgtatccccattttcagctactgatttttcctgtaacacataggaaccaatgctattttgtttagtgttcccatcaggctgacagtcatcacagtttataacagctgaatcactgtcatcaacaccattgacagccaaatagcctgtgatttcttcaactactgcagaattaagtggcccttcctcactgacattcacctttttaatttcccttttctcacaatcatccagtataagacatcgacaagctcgtttagtcccttgaaaatctgcatcattgtccactactgtactcctctgttctactgactccttgtctgattttataggagaatcttcttctgaactgtttggtgcttcagatctaagacaacgcttaattctttttaaaactggtgaaacaggttctgtttgccttctctcacaattttctatagcctgcctttctatgttatccttttctgaagaagaaagtcctcttttcctagggcttacccatgattctcgggtactctgctgttttaaatcagtggttctcccattattatttcctttctgaattggcacaggctctggtctcttctttggtgatcttgatcgtacttgagaattagaagagatttcttcaggatgcgcaatgctacgattccttaaagttctaccacaaaaagattcatccaagccgtttaaccccactgttgatcttgtaacacgagtagatcgggaagcagccatactatggcaagtccctacaatacggtcatcatgatccactcattgggaaaccttttaaaaagcgttttgcctagtatttgatccccatgcgtctgtatttatctgtcatcactgttaattgtccatgttacactgagacttcaggtattatttatttatatggttgtactagaataacttgatatctttcacgcggggtcggacgcaacgggccacttggggaggcgccgccgccgtggccgctctccgcccccgccacggcacttgctcgggtggccaccgctgcaggaagctcgatagcggcgccgcggcgcttccaggt

SEQ ID NO: 18905 - RNA, 881 nt, Homo sapiens
  source 1..881: mol_type = other RNA
tgcctactgagctgatatcagtatttgagcaatccataaaagtcaatcttcaagatgggcaatgacacaggtacttctttagaaatatctttactctgaaacactgagggatcttccttaaatcattccagtagcaaaagccttgccctgaaaaatgttgtcagcagaatagctggaccacccatctggaaccaagttgaagttcatctcttcaaccaaaaaatcctagaatggcccctactgtcagaagatccatgccctccaaatctgaattgatcgtagacactttagctgaagattcctttcttctttaagtatgtccaccaaattctgggccttgcccaagaatcaacaggtaatgtcctttgattccacttgactctgttcggttcaagaaaggggtgcttgcagtcagagtggaccaccacacaactcccgcaactcagtatgccttgaactgctcagagaatggcagttgagcttgtcttcttcactcctggatgtgtactcattccaaaggagtttcacaggcttaacaggaagcacggctgggaggcgtcaggaaacttagaatcatggcagaaggtgaaggggaagcaaggaccttcttcacactcccggcacgagattcaagccagaacttcacaaacattcttttctggttcctcttctttccacacgccacagttagatttgcaaggctgaaattgcctagtgatcatttccattgcagatatcatagacaatgatgcatcttccaggtcagcaatgtggatgataaaactgtctggaacactacattggcaaatgtgagctcatagctaagctgaaatggaaatcagttatgaaacagaactaccagatgccatatgcctgcacac

SEQ ID NO: 18906 - RNA, 68 nt, Homo sapiens
  source 1..68: mol_type = other RNA
tgcctactgagctgatatcagttctcattttacacactggctcagttcagcaggaacaggagtcgagc

SEQ ID NO: 18907 - RNA, 562 nt, Homo sapiens
  source 1..562: mol_type = other RNA
tgcctaggctgagactgcagtgagcagtgatcacatcactacactcaagtctgggcgatgggagtgagactctgtatgtcagtgaaaaatcaccaactattataaaaagaggacaaattgtatcacaaaagaagcaaaaattagaaaaaattcataaaaaaatatatccaactatgaaaagcgttgctctcttggtgtcttcacatccgtctcttctgtgtactgatgtacaacacattgtttcctcggataaatgcatccccatacttattcttcagttgtccatttacatattcttctgtctgctccagggctatattcatgtagccatccaggcaagccaggacccctcgataatccactccagaatttaattttaccacaactggtcgtccgatgatttgctttaagaagtcactaggggtttgcttccgaagactcattttaacaatcctcgccggcgggaaccagaaccctcactccaggcgccccacgagcccggccgccgcggatgatcccagccaaaaccgaaagcgccgaggcaggggcacttttctgcctc

SEQ ID NO: 18908 - RNA, 1256 nt, Homo sapiens
  source 1..1256: mol_type = other RNA
tgcctaggctgagactgcagtgagctgagatcacaccactgcattccagcctgggtgatagagtaagactccatctcaaaataaaaaaaaaaattctcattattctgttcatatcttcctcaacccaaacatccagtgaaaataggtcatcttaataagacggtttgccatgaaaatcatgtccgatcacaccctgcagcctcggcttggccatgaggaggtcaccctcttcttcccttgagtggctttaactccccgggagggtggaatctgcgcccctgtacaagccaggtttccttctcagctcaggagagggacttcttcctgcggatcttgggcttcttcaccggccgcagataagggttatcgatgatgttctcctccccattccggctacccgacaaggaggggttctgctgcaggacagaggtgttctccttctcggctccagaatcctccatgctgatatgaagagcaaggttctctgtgtctgtctgttcatcctgctccgaggaatctgtctcttccatttgttgcatctccagttcagacggaagaagagctgtcaggtaggggatggtgaaaggtctggcagcaatcaatggaaatgtgctgacgtcatctttgaaaagactctgagtctcgcctgtcttggccatgaaacgggtaagtgcccgctccacatcgcgcctctgggatgcagccttctcccgcaggacctggtagtctgacacgggctcacggtacgtcggagttttgatgtaggtgtggggatcagggaactcaggaaaatggctggggatgtgcggcgggtggggtcggttctgccctgcagtgagggccttgggggtcactggctgattggtcaccggaggagcagtgatgaccatcctctgagaccgttttgcataagcagggagagtgtccacattgaaacccatctcaacaagtgtgaccacgatatcggacagtgtgggctgggtcctggctgtgtgctcacagtaagacttggcacttctcccaatttctgaaatgtagctctgcagcatctctgtcagcgtttccacggatgctttctcggcactctcaaaccctgcctctgtcagcaaggagctcacaaccacctgcagggttctcctccgggccagatgatagttatcggcagggttagtggactgtttacttcccgatctcgttccggagccaccggccccagctgtggccgccgcgtcggccatcttgttctggcgtagtgt

SEQ ID NO: 18909 - RNA, 1421 nt, Homo sapiens
  source 1..1421: mol_type = other RNA
tgcctaggctgagactgcagtgagctgagatcacaccactgcattccagcctgggtgatagagtaagactccatctcaaaataaaaaaaaaaattctcattattctgttcatatcttcctcaacccaaacatccagtgaaaataggtcatcttaataagacggtttgccatgaaaatcatgtccgatcacaccctgcagcctcggcttggccatgaggaggtcaccctcttcttcccttgagtggctttaactccccgggagggtggaatctgcgcccctgtacaagccaggtttccttctcagctcaggagagggacttcttcctgcggatcttgggcttcttcaccggccgcagataagggttatcgatgatgttctcctccccattccggctacccgacaaggaggggttctgctgcaggacagaggtgttctccttctcggctccagaatcctccatgctgatatgaagagcaaggttctctgtgtctgtctgttcatcctgctccgaggaatctgtctcttccatttgttgcatctccagttcagacggaagaagagctgtcaggtaggggatggtgaaaggtctggcagcaatcaatggaaatgtgctgacgtcatctttgaaaagactctgagtctcgcctgtcttggccatgaaacgggtaagtgcccgctccacatcgcgcctctgggatgcagccttctcccgcaggacctggtagtctgacacgggctcacggtacgtcggagttttgatgtaggtgtggggatcagggaactcaggaaaatggctggggatgtgcggcgggtggggtcggttctgccctgcagtgagggccttgggggtcactggctgattggtcaccggaggagcagtgatgaccatcctctgagaccgttttgcataagcagggagagtgtccacattgaaacccatctcaacaagtgtgaccacgatatcggacagtgtgggctgggtcctggctgtgtgctcacagtaagacttggcacttctcccaatttctgaaatgtagctctgcagcatctctgtcagcgtttccacggatgctttctcggcactctcaaaccctgcctctgtcagcaaggagctcacaaccacctgcagggttctcctccgggccagatgatagttatcggcagggttagtggactgtttacttcccgatctctaaaacgtacagtcccaatgagataaaatagcaggtcttttactttctactttagcagattattagaatacatagctgaagaaacacgcatgatgggattaagacgtgtcccgcagaaaaaacaggatccctctcttgtgcctcccatcttcacaccatttcattgaaagggaaaatgaaaacagtaacaagaggtgaccgcgaggagaggagggcaaaagataaaa

SEQ ID NO: 18910 - RNA, 965 nt, Homo sapiens
  source 1..965: mol_type = other RNA
tgcctaggctgagactgcagtgagctgagatcacaccactgcattccagcctgggtgatagagtaagactccatctcaaaataaaaaaaaaaattctcattattctgttcatatcttcctcaacccaaacatccagtgaaaataggtcatcttaataagacggtttgccatgaaaatcatgtccgatcacaccctgcagcctcggcttggccatgaggaggtcaccctcttcttcccttgagtggctttaactccccgggagggtggaatctgcgcccctgtacaagccaggtttccttctcagctcaggagagggacttcttcctgcggatcttgggcttcttcaccggccgcagataagggttatcgatgatgttctcctccccattccggctacccgacaaggaggggttctgctgcaggacagaggtgttctccttctcggctccagaatcctccggagttttgatgtaggtgtggggatcagggaactcaggaaaatggctggggatgtgcggcgggtggggtcggttctgccctgcagtgagggccttgggggtcactggctgattggtcaccggaggagcagtgatgaccatcctctgagaccgttttgcataagcagggagagtgtccacattgaaacccatctcaacaagtgtgaccacgatatcggacagtgtgggctgggtcctggctgtgtgctcacagtaagacttggcacttctcccaatttctgaaatgtagctctgcagcatctctgtcagcgtttccacggatgctttctcggcactctcaaaccctgcctctgtcagcaaggagctcacaaccacctgcagggttctcctccgggccagatgatagttatcggcagggttagtggactgtttacttcccgatctcgttccggagccaccggccccagctgtggccgccgcgtcggccatcttgttctggcgtagtgt

SEQ ID NO: 18911 - RNA, 1380 nt, Homo sapiens
  source 1..1380: mol_type = other RNA
tgcctaggctgagactgcagtgagctgagatcacaccactgcattccagcctgggtgatagagtaagactccatctcaaaataaaaaaaaaaattctcattattctgttcatatcttcctcaacccaaacatccagtgaaaataggtcatcttaataagacggtttgccatgaaaatcatgtccgatcacaccctgcagcctcggcttggccatgaggaggtcaccctcttcttcccttgagtggctttaactccccgggagggtggaatctgcgcccctgtacaagccaggtttccttctcagctcaggagagggacttcttcctgcggatcttgggcttcttcaccggccgcagataagggttatcgatgatgttctcctccccattccggctacccgacaaggaggggttctgctgcaggacagaggtgttctccttctcggctccagaatcctcctgtaattccagctactcaggaggctgaggctggagaatcgcttgaacccaggaggcggaggttgcagtgagccaagatcttgccactgcactccagcctgggtgacggagcgagactctatcatgctgatatgaagagcaaggttctctgtgtctgtctgttcatcctgctccgaggaatctgtctcttccatttgttgcatctccagttcagacggaagaagagctgtcaggtaggggatggtgaaaggtctggcagcaatcaatggaaatgtgctgacgtcatctttgaaaagactctgagtctcgcctgtcttggccatgaaacgggtaagtgcccgctccacatcgcgcctctgggatgcagccttctcccgcaggacctggtagtctgacacgggctcacggtacgtcggagttttgatgtaggtgtggggatcagggaactcaggaaaatggctggggatgtgcggcgggtggggtcggttctgccctgcagtgagggccttgggggtcactggctgattggtcaccggaggagcagtgatgaccatcctctgagaccgttttgcataagcagggagagtgtccacattgaaacccatctcaacaagtgtgaccacgatatcggacagtgtgggctgggtcctggctgtgtgctcacagtaagacttggcacttctcccaatttctgaaatgtagctctgcagcatctctgtcagcgtttccacggatgctttctcggcactctcaaaccctgcctctgtcagcaaggagctcacaaccacctgcagggttctcctccgggccagatgatagttatcggcagggttagtggactgtttacttcccgatctcgttccggagccaccggccccagctgtggccgccgcgtcggccatcttgttctggcgtagtgtgc

SEQ ID NO: 18912 - RNA, 5084 nt, Homo sapiens
  source 1..5084: mol_type = other RNA
tgcctaggctgagactgcagtgcagtggcacaatcatggcccactgtagctttgaactccttggttcaaagtattcaaggtatgatcgaattaaacttcttccctcaaatcttcccaattccccaagtcagaatttattcattcattcatcaaatactgaacaagcacctattatgtgctaggtactctactaggttgtctgagctacgttgtagttctgataacattatagaacttctcatcccttcctatagtcattaatatttgcatatgcaatttcttccttccttaactgtgtgcttctagagtgatggaactgtgtccagttcacctctgtaacccaggcatctggacaatgctttggaaatagtaattaaaatgaaatacaagagtgccaaaacaaactccaagtggctagaagaaaaatgtctcctaaaccatctgggtttgctaaacataaccagaaagacaacagtacctgatgataatcagttgtcttataaataacaccagatcacaattaattagcttcttttatgcttttttctattcttgttggaaaatgtattgacaactattttttaatcccttatttaaaggatactaataagtcagtggtccatatttcagttacatgtacatcaaaaccagttagcaagaaaaatgaaaatacactcaagtgattttcagaaacataaaaatcaccatcaccaaccaccccaaaccaggaaacacttcctccttcactcactgccacaaacccagttacagcaacagtaagaattgacagcgataaaataaagagcccaaaaggaatgaaaaaactcagaaagtgccatgtataagaaaaaaaaggttcaaatgtgtttggcaaactaatgtcccaggatcccagttccaaactaagcaaaattcatgggcagaataaacatagaatgtggtcaaatccattgagagattaaaagcttttctgaggtcaagaaaccttaggttacaacgaaggttattcaaagggaactagggctttattattcaaagggaactaggctttcaaagaagaagaaaatgatcaaggtacccacaagctccaggcccatggttggtacttaataaatgagagctattatgaggagctgagaactaactcaaatgtccctcttttgtgatgtctcagggaggatcactgaatatctttctctgtgctcccatagtactctatacaggctgctatcatatcatttactgtatgtactagggtccgaatgctgtgtccctcctaaattcacatgttgaaatataatgtttaatgtggtgatatctggagacggggcctgtgggaggtaatttggtcataaggatggaatcctcatgaatgggattagtgcccttataaaaagaggccagagaattagcttgcactcttttcaccatctggggataaagtgacaagtcagcagtttgaaacctggaagagggccctcaccataacctatggtggtactttgatcttgaacttccagactacagaatgtgagaaataaattactgtgtttataagccatccagtctatggtattttgtaattgcagcctggactgagacaatatgtcatctatattatgacatatgacatctatacatatgcagaaccaagattctttctttaagtcttcttgttcattccctcacatttcaaatgccattctctttcattacttgttctgttcaaagtaatgtctcttattccactaccaacatagaataagcttcatggagtaaattcttccagatgatgcagtatgaaatgataggagagcatgaagttattttttttcattcttgttttgaaataattttaagtaaacaaatatgttgcaaaaatagagcattcctttaacccagtgtcccttactgttaacatcttacaaaaacatagtataataattgaaaggaggaaattaacattgagccaataaaacagactattctatagatcttacttgaatttccaagttttcccattgatgtcctttttctggtccaggatcatacattacatttaattgttatgtgtccttagtctcctccattctgtgacagttcctcactttttccttgtcgtcaactggtgtatcaggaggtccattaagaaggtaatcttgttactaaacagaacatcactgcagttttctgaacagttattgcaggtgaggttgtaaacattgattgcattgcagagagacttaggaggaattcttaaaactgtgttcacatttgtggctgggactactgcttgaaggatgtgttcaagggctgttaatccaccagcagcttgaaatgcaatctgatctgccacattctctttttccagtattctagtgatctctcctagggtccgatccaaagcagacactttattgtttgcccatgagccactgtcttgaacttgtacttgttttagaagatctttggctaatcgctgaagctttgctttataaggtgaatcagagccagaatttttggtttccattaaactctcatattccttagccctgaagttcatccgggcttttatctttttggctttttttttatttttttgccgctcttctccatctttcaaagcttctgctggagctgtactttcaaccacaatgtcaataatgtacttcttcaaggaaagatgctccacttcttcatctgacagttcacgcccctggatgctggtattctctctcacggcttgctggtgttttctccctttaacatggctaaaaagatatacctctgaagagatcaggacattgcagagagaacactgcttctttctttcataaggggtcagtttgggggcataatcagtatttgcatgtcgcccactgcttagctcagcagctttttcttttctttgttcaatctgttccatgtgccttcgaatactttcatcatgcttgagctgaatttttttctgtaactcttccatagcttcttgttgagcagctgtgagtgctgccaatcgttcttccctgtctctagctctttcccgggctgcatcctcacgggctttttccttttcttgcctctgttgttcaattcgggcttcttgttctttcctcttcattaacaattcttctacacgggcctgccgctctgcctctagagctctcttgcgttcctgcacagcttcatcacgtgcttgcttttcttcctgtcttctctgacgctcttcctgtagctcattaagcctctgttcatattccttcaattttgataaaacatcatgacgtttattctgggcttcaagggtatttataaaggcaatttcatttaccttagcttcttcttcttgtgcttttttcacaattgcttgtaactgcacttctcgcttaaactcagcatgaagtaatttttcttccatcatcctgcgtcgttgatctagcaattcttccttccacttccggacatccttctccctttctaacaatttctgaagcttcaatgttttctcttcgcgtaacttttcccttagctgctgtgctttcatttgtttttcttcatgtttcttcttagattctgcaattgttcttttacgagagggtgaagaaagtttttcatgcatgtgaattccatgccctggaggtctagcaggttcttcttctacaatgtccccccaggatgtattttggcgccaagactcacgagcttcataatctgcaaggacatcgttccagtccatggacataccacagaaagaaacactcccactgcccatgctggcagaaaaatcactgtcgttgtcagtttcaatgttaatatcattgttttcttcagcttcaatttctctagttaactgttcttcttcagcaatagcactagcaatggcttcttcattggccttttctagacgatctgctagctcttcttttttagcaaggacttctgccatggacaagttagcagcactcacatttgaaatatctgaagggtccatttcattttctatccttgctttctctgctggaaatttttcttcatttacttgtaaaggaggtgtaccagcttgcagcataactgaaacacactctgtatcaatgtggacagcagatatttcagaagttcgaacataattgtctcgaatactgccagaattcttcacatcatccaatgtactcactgtgaactgggttttttcggcaagaggatggtcacaagagtgtaatgagtctttgggatgagattctatagtattagaagttccatctccaacaaattgacctttctgtatgctttcatcaggtaaaagacatacattttctttatcactgtcatcctttgatcttgtggcttctgttgccaatgaaacttttggcatcactgctgttgatcgagaacgaataggccttcctctctgaacggtctcccatccttcagcatctttccgttcatttttgcgtgaggccttctgcactgtcattggtgggcaagactgggcgggtgttatttctgaagaagcagtagagcctgtatgatgagcctttaccttgtcagcccaactgacacctgtgggagccagacgaggagctggcactgtgccagttgaacctccaaaatttaagcttcgtcgagcatttgatgttacatttattctatctgttgatggacttggaatcacatggcgtcccggagacatcttctttacttcccatgccaatgatgttggtctgctttgagcatctgtcttctctagcttttcctgaagctgaatccagtcaatcaatgctttgaaatctcttacatagttatccagcatcattagcacctccttacattcgaccacactctgatctgattcgcaagttacatagatttcatctactgctcggcgaagattatcaaaaagaaatgcccagtatcgagctcttagatcaattttccgagggtgccttgttttagtgggacttttatcaaagtgtttatctccagtcgtagacgatgttattttacagtccactgcagtactctgtttagtagttttatgagtgccttgaatggtcctcttagattttccaccagtttgacattta

SEQ ID NO: 18913 - RNA, 5243 nt, Homo sapiens
  source 1..5243: mol_type = other RNA
tgcctaggctgagactgcagtgcagtggcacaatcatggcccactgtagctttgaactccttggttcaaagtattcaaggtatgatcgaattaaacttcttccctcaaatcttcccaattccccaagtcagaatttattcattcattcatcaaatactgaacaagcacctattatgtgctaggtactctactaggttgtctgagctacgttgtagttctgataacattatagaacttctcatcccttcctatagtcattaatatttgcatatgcaatttcttccttccttaactgtgtgcttctagagtgatggaactgtgtccagttcacctctgtaacccaggcatctggacaatgctttggaaatagtaattaaaatgaaatacaagagtgccaaaacaaactccaagtggctagaagaaaaatgtctcctaaaccatctgggtttgctaaacataaccagaaagacaacagtacctgatgataatcagttgtcttataaataacaccagatcacaattaattagcttcttttatgcttttttctattcttgttggaaaatgtattgacaactattttttaatcccttatttaaaggatactaataagtcagtggtccatatttcagttacatgtacatcaaaaccagttagcaagaaaaatgaaaatacactcaagtgattttcagaaacataaaaatcaccatcaccaaccaccccaaaccaggaaacacttcctccttcactcactgccacaaacccagttacagcaacagtaagaattgacagcgataaaataaagagcccaaaaggaatgaaaaaactcagaaagtgccatgtataagaaaaaaaaggttcaaatgtgtttggcaaactaatgtcccaggatcccagttccaaactaagcaaaattcatgggcagaataaacatagaatgtggtcaaatccattgagagattaaaagcttttctgaggtcaagaaaccttaggttacaacgaaggttattcaaagggaactagggctttattattcaaagggaactaggctttcaaagaagaagaaaatgatcaaggtacccacaagctccaggcccatggttggtacttaataaatgagagctattatgaggagctgagaactaactcaaatgtccctcttttgtgatgtctcagggaggatcactgaatatctttctctgtgctcccatagtactctatacaggctgctatcatatcatttactgtatgtactagggtccgaatgctgtgtccctcctaaattcacatgttgaaatataatgtttaatgtggtgatatctggagacggggcctgtgggaggtaatttggtcataaggatggaatcctcatgaatgggattagtgcccttataaaaagaggccagagaattagcttgcactcttttcaccatctggggataaagtgacaagtcagcagtttgaaacctggaagagggccctcaccataacctatggtggtactttgatcttgaacttccagactacagaatgtgagaaataaattactgtgtttataagccatccagtctatggtattttgtaattgcagcctggactgagacaatatgtcatctatattatgacatatgacatctatacatatgcagaaccaagattctttctttaagtcttcttgttcattccctcacatttcaaatgccattctctttcattacttgttctgttcaaagtaatgtctcttattccactaccaacatagaataagcttcatggagtaaattcttccagatgatgcagtatgaaatgataggagagcatgaagttattttttttcattcttgttttgaaataattttaagtaaacaaatatgttgcaaaaatagagcattcctttaacccagtgtcccttactgttaacatcttacaaaaacatagtataataattgaaaggaggaaattaacattgagccaataaaacagactattctatagatcttacttgaatttccaagttttcccattgatgtcctttttctggtccaggatcatacattacatttaattgttatgtgtccttagtctcctccattctgtgacagttcctcactttttccttgtctttcatgatattgacgtttttgaaaaatattagtcagttattgtgcagaatgtcccccaacttgggtatgatacacctaggtctgattcttggctttctgacttaatatctatgtagccttgggcaagtcaacctctctgggactcaagtttcctcatcgtcaactggtgtatcaggaggtccattaagaaggtaatcttgttactaaacagaacatcactgcagttttctgaacagttattgcaggtgaggttgtaaacattgattgcattgcagagagacttaggaggaattcttaaaactgtgttcacatttgtggctgggactactgcttgaaggatgtgttcaagggctgttaatccaccagcagcttgaaatgcaatctgatctgccacattctctttttccagtattctagtgatctctcctagggtccgatccaaagcagacactttattgtttgcccatgagccactgtcttgaacttgtacttgttttagaagatctttggctaatcgctgaagctttgctttataaggtgaatcagagccagaatttttggtttccattaaactctcatattccttagccctgaagttcatccgggcttttatctttttggctttttttttatttttttgccgctcttctccatctttcaaagcttctgctggagctgtactttcaaccacaatgtcaataatgtacttcttcaaggaaagatgctccacttcttcatctgacagttcacgcccctggatgctggtattctctctcacggcttgctggtgttttctccctttaacatggctaaaaagatatacctctgaagagatcaggacattgcagagagaacactgcttctttctttcataaggggtcagtttgggggcataatcagtatttgcatgtcgcccactgcttagctcagcagctttttcttttctttgttcaatctgttccatgtgccttcgaatactttcatcatgcttgagctgaatttttttctgtaactcttccatagcttcttgttgagcagctgtgagtgctgccaatcgttcttccctgtctctagctctttcccgggctgcatcctcacgggctttttccttttcttgcctctgttgttcaattcgggcttcttgttctttcctcttcattaacaattcttctacacgggcctgccgctctgcctctagagctctcttgcgttcctgcacagcttcatcacgtgcttgcttttcttcctgtcttctctgacgctcttcctgtagctcattaagcctctgttcatattccttcaattttgataaaacatcatgacgtttattctgggcttcaagggtatttataaaggcaatttcatttaccttagcttcttcttcttgtgcttttttcacaattgcttgtaactgcacttctcgcttaaactcagcatgaagtaatttttcttccatcatcctgcgtcgttgatctagcaattcttccttccacttccggacatccttctccctttctaacaatttctgaagcttcaatgttttctcttcgcgtaacttttcccttagctgctgtgctttcatttgtttttcttcatgtttcttcttagattctgcaattgttcttttacgagagggtgaagaaagtttttcatgcatgtgaattccatgccctggaggtctagcaggttcttcttctacaatgtccccccaggatgtattttggcgccaagactcacgagcttcataatctgcaaggacatcgttccagtccatggacataccacagaaagaaacactcccactgcccatgctggcagaaaaatcactgtcgttgtcagtttcaatgttaatatcattgttttcttcagcttcaatttctctagttaactgttcttcttcagcaatagcactagcaatggcttcttcattggccttttctagacgatctgctagctcttcttttttagcaaggacttctgccatggacaagttagcagcactcacatttgaaatatctgaagggtccatttcattttctatccttgctttctctgctggaaatttttcttcatttacttgtaaaggaggtgtaccagcttgcagcataactgaaacacactctgtatcaatgtggacagcagatatttcagaagttcgaacataattgtctcgaatactgccagaattcttcacatcatccaatgtactcactgtgaactgggttttttcggcaagaggatggtcacaagagtgtaatgagtctttgggatgagattctatagtattagaagttccatctccaacaaattgacctttctgtatgctttcatcaggtaaaagacatacattttctttatcactgtcatcctttgatcttgtggcttctgttgccaatgaaacttttggcatcactgctgttgatcgagaacgaataggccttcctctctgaacggtctcccatccttcagcatctttccgttcatttttgcgtgaggccttctgcactgtcattggtgggcaagactgggcgggtgttatttctgaagaagcagtagagcctgtatgatgagcctttaccttgtcagcccaactgacacctgtgggagccagacgaggagctggcactgtgccagttgaacctccaaaatttaagcttcgtcgagcatttgatgttacatttattctatctgttgatggacttggaatcacatggcgtcccggagacatcttctttacttcccatgccaatgatgttggtctgctttgagcatctgtcttctctagcttttcctgaagctgaatccagtcaatcaatgctttgaaatctcttacatagttatccagcatcattagcacctccttacattcgaccacactctgatctgattcgcaagttacatagatttcatctactgctcggcgaagattatcaaaaagaaatgcccagtatcgagctcttagatcaattttccgagggtgccttgttttagtgggacttttatcaaagtgtttatctccagtcgtagacgatgttattttacagtccactgcagtactctgtttagtagttttatgagtgccttgaatggtcctcttagattttccaccagtttgacattta

SEQ ID NO: 18914 - RNA, 3918 nt, Homo sapiens
  source 1..3918: mol_type = other RNA
tgcctccttggtctccggcagcagcataatgctgagaatgcagaggagggcgcaggccgccagcaccacgtgctgcaggaaggctccatggcccatgtggaggcgctgggccgggccgctcagtcctccaagcgcccctagagccatgatcaggcccaggccacggccccggacagtggtggggatgacctcagcagcaaggagggtgctgaggatggcggcagcttgggaggagaagagcccaaggacagagaaagtggtgatggcagcctcgttcagataatcccacaggcccagcaggaccagggaagcaatgccggtaagggtcatggagagaagaaggatgccccggcggccaaatcggtccacggtgacccccaggaagacacaggccagggctgcggtgccgctggccagcagagagcacaggtagaagtccgatgggctccctcctcctcccacaggctggtagcagtggcgaatggcatgggcaatgaagcctgcagggcctcctgggcctcctcccccagcatctgcccatggggccggtttcgctcagccaggatcctcagcacagactgagcctcctcaatctgccgcttcactatcagccaccgtgcggactccaggaacaaaccaggccagccataaaacaggaagaggatgcagggagcggtgatcattcgctgtaggaatcgccaatccttagagacaagggccaggcccaggaacaggaagtgccctcccacccccaccaactcccctgccagggccacccgaagcctctgggttgggtcgcacagctccaggcgcatcaggtagacacccaggtcaacaccggcaagcagaaagcccaagaggaatcggagggccatgacgcctgtggaggagcctgcagcagcccctcctactccacaggggcccaccagccccaaggtcagcagcacaatcccgcgacggccaaatctgtctgcggggtaacccaggaacaggtagccggaggcaaagcccaagatgaagaggatctgctccaggatcacctgccagcccaggtcacacaccagatcccactggccgatggcgttggtggtgagcacaggaaggccattatagtcccaatccttgaggcaatggttgaagtccggcggggcgaagccgctgcacgaggggtcggtactggtggcgacacggctggcggcgctggctgctagggcagcgctggcgacgctgacgccgctggcattgggaggctgctcccagccagaggcattaggggggaaggccccgtagtggcaatgcagcgggggcgccagcgtgaagatggggtccgaggccatgcccagagccacgaagagcaccggcaggcagcagaggccgagctgcagctgctggccgccgcccagcgcccccacctgggcgagcagcgcctcaaagctgagggggcctgggggcacggccagcgacaggctgctgcccagtccgtcgccgcccgcgtctccctccccctcccgctcgcgctcccgctcaccctgcagctgctccgtgggcaccgcatctccgagggtcccgacctgtccgttggaggtgggggtgatctctacagtgttgtcgattttgccgccgcccccgccattgggctcgggggtcccggtggccacccggggagccagcttgccgaccgcaggggccctgccggcccgcgccgaaaggatgcgctgtcctctggctcagttgcgcgccggctgcccggacacagacagctcgaagagatcccgctctgcagctctgcagccgcgggcgcctccttggtctctgcgatctctgcgctgctttcccctccccttcctctagactctcctccccttcccacgtcagcagaaccttcggtccagactcttcgtcagagagaggaaggggggccagggcccaggggagggagggaaggggggctctgtcgtctctttcctgggtctgcgggccattgcggtaaaaaagaaaaaaagctgaaggatagtagctagtccaggcagatgccagagattcttcctctgcttccaatcatttgccatcattcattcattcattcattcacccattcactaatcagtaaaatttaagtgtccactacgttccaggacttgcactagactttaaggataacagggtggacaagttccactttggagacctttactccagggagacagacatgtaaactggctattacagtacaacttatgcatatggaagactgtcttggccctgtatcagccctagcttcagtcctctacaaggagaccactttcttgggtttcatcactcccatcctgtttgaatctccatttctcaacagcatttggcactgttgacccctcttcctctaaacactctcttcctttgctgctgagtctctcttgctccccttttctccattgcagaaatcgtcttccagctcatggcattggtgctgagcatgggcaggccattatcctcccggttcttgaggcaatgattgaagtccagcggggtgacgcaactgcaggaggggtctgtattggtagtgatgaggctgtggtgctggcttctagggccattcccgtctgtatcatttagacaccatggttcagtgtctggaatcctcacagacttagtcctaggccctcctctcatctcacactgtctccactttgggatcttacctatgcccacagcttcaatcaccacccatacaaacaatacaaacctgacgcccagactgacatctccagcttccacctctgttctgagctccagacctatgaagccacctcttatttgaccttcaccttggatgactcacagggacctcaaactcaatatgttcaagacgaaatttttgcttttcccccataacttggttggcttccactgcttttttctgcagcgaatggcaccctcaacatcgcattgtggccaaatgctcaggcaacagcctttagagctttctcttccttatccatgttgaattctttacaaaattctgcccattttacttcctatatattctcagacatcccacatctctccatctctaccattattagtcaagctacctgttgcaaagaccactttagctccctaattcctaactggtgttcagcgtccgctttgtttatacctccttatcacccatatgtcatttatagtcagatagaatgatcttttcaaaatacagatctgatcatgtatctttcctgctaaccagccttcagtggtgtctcctcactgtcaaagtgaatattaaaaatctagatacctcatacatggttctacatgcctggtcacatgctgtctgtagttccatctcacttctttccccaaactctctgcactccagccacagaccttcttctagttttcccagcgccacgaggcctttgaacaagctggttcctgcacctaaaaagcttcttagtcacatttttctcatccttcagctctcagcctaaacatctttgctacacaggagtcttccctaacctctagaattgctactcaaagtgtggttcatggaccagcagcattcctgggagcttgttagaaatgcagaatccaagcctcacccagacccttgaatcataatctgtattttatccagatctccaggcataggtattatacattaaaggtagagacacacatctctaagagatttgttacctgataggtactttattctctaatcctaggtaagggctagaaagcagtgttctatcattgtcagccgggaaatctttcccccttctctccactgaaccacacttttaacttgtctctgttcagaaattttccacgtatgggaaactcttttcttcagacagggtctcactgtcttacccaggatggagtgcagtggcttgatcacagctcactgcagtc

SEQ ID NO: 18915 - RNA, 3915 nt, Homo sapiens
  source 1..3915: mol_type = other RNA
tgcctccttggtctccggcagcagcataatgctgagaatgcagaggagggcgcaggccgccagcaccacgtgctgcaggaaggctccatggcccatgtggaggcgctgggccgggccgctcagtcctccaagcgcccctagagccatgatcaggcccaggccacggccccggacagtggtggggatgacctcagcagcaaggagggtgctgaggatggcggcagcttgggaggagaagagcccaaggacagagaaagtggtgatggcagcctcgttcagataatcccacaggcccagcaggaccagggaagcaatgccggtaagggtcatggagagaagaaggatgccccggcggccaaatcggtccacggtgacccccaggaagacacaggccagggctgcggtgccgctggccagcagagagcacaggtagaagtccgatgggctccctcctcctcccacaggctggtagcagtggcgaatggcatgggcaatgaagcctgcagggcctcctgggcctcctcccccagcatctgcccatggggccggtttcgctcagccaggatcctcagcacagactgagcctcctcaatctgccgcttcactatcagccaccgtgcggactccaggaacaaaccaggccagccataaaacaggaagaggatgcagggagcggtgatcattcgctgtaggaatcgccaatccttagagacaagggccaggcccaggaacaggaagtgccctcccacccccaccaactcccctgccagggccacccgaagcctctgggttgggtcgcacagctccaggcgcatcaggtagacacccaggtcaacaccggcaagcagaaagcccaagaggaatcggagggccatgacgcctgtggaggagcctgcagcagcccctcctactccacaggggcccaccagccccaaggtcagcagcacaatcccgcgacggccaaatctgtctgcggggtaacccaggaacaggtagccggaggcaaagcccaagatgaagaggatctgctccaggatcacctgccagcccaggtcacacaccagatcccactggccgatggcgttggtggtgagcacaggaaggccattatagtcccaatccttgaggcaatggttgaagtccggcggggcgaagccgctgcacgaggggtcggtactggtggcgacacggctggcggcgctggctgctagggcagcgctggcgacgctgacgccgctggcattgggaggctgctcccagccagaggcattaggggggaaggccccgtagtggcaatgcagcgggggcgccagcgtgaagatggggtccgaggccatgcccagagccacgaagagcaccggcaggcagcagaggccgagctgcagctgctggccgccgcccagcgcccccacctgggcgagcagcgcctcaaagctgagggggcctgggggcacggccagcgacaggctgctgcccagtccgtcgccgcccgcgtctccctccccctcccgctcgcgctcccgctcaccctgcagctgctccgtgggcaccgcatctccgagggtcccgactccgttggaggtgggggtgatctctacagtgttgtcgattttgccgccgcccccgccattgggctcgggggtcccggtggccacccggggagccagcttgccgaccgcaggggccctgccggcccgcgccgaaaggatgcgctgtcctctggctcagttgcgcgccggctgcccggacacagacagctcgaagagatcccgctctgcagctctgcagccgcgggcgcctccttggtctctgcgatctctgcgctgctttcccctccccttcctctagactctcctccccttcccacgtcagcagaaccttcggtccagactcttcgtcagagagaggaaggggggccagggcccaggggagggagggaaggggggctctgtcgtctctttcctgggtctgcgggccattgcggtaaaaaagaaaaaaagctgaaggatagtagctagtccaggcagatgccagagattcttcctctgcttccaatcatttgccatcattcattcattcattcattcacccattcactaatcagtaaaatttaagtgtccactacgttccaggacttgcactagactttaaggataacagggtggacaagttccactttggagacctttactccagggagacagacatgtaaactggctattacagtacaacttatgcatatggaagactgtcttggccctgtatcagccctagcttcagtcctctacaaggagaccactttcttgggtttcatcactcccatcctgtttgaatctccatttctcaacagcatttggcactgttgacccctcttcctctaaacactctcttcctttgctgctgagtctctcttgctccccttttctccattgcagaaatcgtcttccagctcatggcattggtgctgagcatgggcaggccattatcctcccggttcttgaggcaatgattgaagtccagcggggtgacgcaactgcaggaggggtctgtattggtagtgatgaggctgtggtgctggcttctagggccattcccgtctgtatcatttagacaccatggttcagtgtctggaatcctcacagacttagtcctaggccctcctctcatctcacactgtctccactttgggatcttacctatgcccacagcttcaatcaccacccatacaaacaatacaaacctgacgcccagactgacatctccagcttccacctctgttctgagctccagacctatgaagccacctcttatttgaccttcaccttggatgactcacagggacctcaaactcaatatgttcaagacgaaatttttgcttttcccccataacttggttggcttccactgcttttttctgcagcgaatggcaccctcaacatcgcattgtggccaaatgctcaggcaacagcctttagagctttctcttccttatccatgttgaattctttacaaaattctgcccattttacttcctatatattctcagacatcccacatctctccatctctaccattattagtcaagctacctgttgcaaagaccactttagctccctaattcctaactggtgttcagcgtccgctttgtttatacctccttatcacccatatgtcatttatagtcagatagaatgatcttttcaaaatacagatctgatcatgtatctttcctgctaaccagccttcagtggtgtctcctcactgtcaaagtgaatattaaaaatctagatacctcatacatggttctacatgcctggtcacatgctgtctgtagttccatctcacttctttccccaaactctctgcactccagccacagaccttcttctagttttcccagcgccacgaggcctttgaacaagctggttcctgcacctaaaaagcttcttagtcacatttttctcatccttcagctctcagcctaaacatctttgctacacaggagtcttccctaacctctagaattgctactcaaagtgtggttcatggaccagcagcattcctgggagcttgttagaaatgcagaatccaagcctcacccagacccttgaatcataatctgtattttatccagatctccaggcataggtattatacattaaaggtagagacacacatctctaagagatttgttacctgataggtactttattctctaatcctaggtaagggctagaaagcagtgttctatcattgtcagccgggaaatctttcccccttctctccactgaaccacacttttaacttgtctctgttcagaaattttccacgtatgggaaactcttttcttcagacagggtctcactgtcttacccaggatggagtgcagtggcttgatcacagctcactgcagtc

SEQ ID NO: 18916 - RNA, 1587 nt, Homo sapiens
  source 1..1587: mol_type = other RNA
tgcctccttggtctccggcagcagcataatgctgagaatgcagaggagggcgcaggccgccagcaccacgtgctgcaggaaggctccatggcccatgtggaggcgctgggccgggccgctcagtcctccaagcgcccctagagccatgatcaggcccaggccacggccccggacagtggtggggatgacctcagcagcaaggagggtgctgaggatggcggcagcttgggaggagaagagcccaaggacagagaaagtggtgatggcagcctcgttcagataatcccacaggcccagcaggaccagggaagcaatgccggtaagggtcatggagagaagaaggatgccccggcggccaaatcggtccacggtgacccccaggaagacacaggccagggctgcggtgccgctggccagcagagagcacaggtagaagtccgatgggctccctcctcctcccacaggctggtagcagtggcgaatggcatgggcaatgaagcctgcagggcctcctgggcctcctcccccagcatctgcccatggggccggtttcgctcagccaggatcctcagcacagactgagcctcctcaatctgccgcttcactatcagccaccgtgcggactccaggaacaaaccaggccagccataaaacaggaagaggatgcagggagcggtgatcattcggcatcaggtagacacccaggtcaacaccggcaagcagaaagcccaagaggaatcggagggccatgacgcctgtggaggagcctgcagcagcccctcctactccacaggggcccaccagccccaaggtcagcagcacaatcccgcgacggccaaatctggccgatggcgttggtggtgagcacaggaaggccattatagtcccaatccttgaggcaatggttgaagtccggcggggcgaagccgctgcacgaggggtcggtactggtggcgacacggctggcggcgctggctgctagggcagcgctggcgacgctgacgccgctggcattgggaggctgctcccagccagaggcattaggggggaaggccccgtagtggcaatgcagcgggggcgccagcgtgaagatggggtccgaggccatgcccagagccacgaagagcaccggcaggcagcagaggccgagctgcagctgctggccgccgcccagcgcccccacctgggcgagcagcgcctcaaagctgagggggcctgggggcacggccagcgacaggctgctgcccagtccgtcgccgcccgcgtctccctccccctcccgctcgcgctcccgctcaccctgcagctgctccgtgggcaccgcatctccgagggtcccgacctgtccgttggaggtgggggtgatctctacagtgttgtcgattttgccgccgcccccgccattgggctcgggggtcccggtggccacccggggagccagcttgccgaccgcaggggccctgccggcccgcgccgaaaggatgcgctgtcctctggctcagttgcgcgccggctgcccggacacagacagctcgaagagatcccgctctgcagctctgcagccgcgggcgcctccttggtctctgc

SEQ ID NO: 18917 - RNA, 1922 nt, Homo sapiens
  source 1..1922: mol_type = other RNA
tgcctccttggtctccggcagcagcataatgctgagaatgcagaggagggcgcaggccgccagcaccacgtgctgcaggaaggctccatggcccatgtggaggcgctgggccgggccgctcagtcctccaagcgcccctagagccatgatcaggcccaggccacggccccggacagtggtggggatgacctcagcagcaaggagggtgctgaggatggcggcagcttgggaggagaagagcccaaggacagagaaagtggtgatggcagcctcgttcagataatcccacaggcccagcaggaccagggaagcaatgccggtaagggtcatggagagaagaaggatgccccggcggccaaatcggtccacggtgacccccaggaagacacaggccagggctgcggtgccgctggccagcagagagcacaggtagaagtccgatgggctccctcctcctcccacaggctggtagcagtggcgaatggcatgggcaatgaagttggtgaagcccaggataagcagatttttccagatgttgcggtagttgaggagggaagcaaaggaaaaggaggatgttgcagggagagggcaggtattctccaggtcctgcagggcctcctgggcctcctcccccagcatctgcccatggggccggtttcgctcagccaggatcctcagcacagactgagcctcctcaatctgccgcttcactatcagccaccgtgcggactccaggaacaaaccaggccagccataaaacaggaagaggatgcagggagcggtgatcattcgctgtaggaatcgccaatccttagagacaagggccaggcccaggaacaggaagtgccctcccacccccaccaactcccctgccagggccacccgaagcctctgggttgggtcgcacagctccaggcgcatcaggtagacacccaggtcaacaccggcaagcagaaagcccaagaggaatcggagggccatgacgcctgtggaggagcctgcagcagcccctcctactccacaggggcccaccagccccaaggtcagcagcacaatcccgcgacggccaaatctgtctgcggggtaacccaggaacaggtagccggaggcaaagcccaagatgaagaggatctgctccaggatcacctgccagcccaggtcacacaccagatcccactggccgatggcgttggtggtgagcacaggaaggccattatagtcccaatccttgaggcaatggttgaagtccggcggggcgaagccgctgcacgaggggtcggtactggtggcgacacggctggcggcgctggctgctagggcagcgctggcgacgctgacgccgctggcattgggaggctgctcccagccagaggcattaggggggaaggccccgtagtggcaatgcagcgggggcgccagcgtgaagatggggtccgaggccatgcccagagccacgaagagcaccggcaggcagcagaggccgagctgcagctgctggccgccgcccagcgcccccacctgggcgagcagcgcctcaaagctgagggggcctgggggcacggccagcgacaggctgctgcccagtccgtcgccgcccgcgtctccctccccctcccgctcgcgctcccgctcaccctgcagctgctccgtgggcaccgcatctccgagggtcccgacctgtccgttggaggtgggggtgatctctacagtgttgtcgattttgccgccgcccccgccattgggctcgggggtcccggtggccacccggggagccagcttgccgaccgcaggggccctgccggcccgcgccgaaaggatgcgctgtcctctggctcagttgcgcgccggctgcccggacacagacagctcgaagagatcccgctctgcagctctgcagccgcgggcgcctccttggtctctgc

SEQ ID NO: 18918 - RNA, 4019 nt, Homo sapiens
  source 1..4019: mol_type = other RNA
tgcctccttggtctccggcagcagcataatgctgagaatgcagaggagggcgcaggccgccagcaccacgtgctgcaggaaggctccatggcccatgtggaggcgctgggccgggccgctcagtcctccaagcgcccctagagccatgatcaggcccaggccacggccccggacagtggtggggatgacctcagcagcaaggagggtgctgaggatggcggcagcttgggaggagaagagcccaaggacagagaaagtggtgatggcagcctcgttcagataatcccacaggcccagcaggaccagggaagcaatgccggtaagggtcatggagagaagaaggatgccccggcggccaaatcggtccacggtgacccccaggaagacacaggccagggctgcggtgccgctggccagcagagagcacaggtagaagtccgatgggctccctcctcctcccacaggctggtagcagtggcgaatggcatgggcaatgaagttggtgaagcccaggataagcagatttttccagatgttgcggtagttgaggagggaagcaaaggaaaaggaggatgttgcagggagagggcaggtattctccaggtcctgcagggcctcctgggcctcctcccccagcatctgcccatggggccggtttcgctcagccaggatcctcagcacagactgagcctcctcaatctgccgcttcactatcagccaccgtgcggactccaggaacaaaccaggccagccataaaacaggaagaggatgcagggagcggtgatcattcgctgtaggaatcgccaatccttagagacaagggccaggcccaggaacaggaagtgccctcccacccccaccaactcccctgccagggccacccgaagcctctgggttgggtcgcacagctccaggcgcatcaggtagacacccaggtcaacaccggcaagcagaaagcccaagaggaatcggagggccatgacgcctgtggaggagcctgcagcagcccctcctactccacaggggcccaccagccccaaggtcagcagcacaatcccgcgacggccaaatctgtctgcggggtaacccaggaacaggtagccggaggcaaagcccaagatgaagaggatctgctccaggatcacctgccagcccaggtcacacaccagatcccactggccgatggcgttggtggtgagcacaggaaggccattatagtcccaatccttgaggcaatggttgaagtccggcggggcgaagccgctgcacgaggggtcggtactggtggcgacacggctggcggcgctggctgctagggcagcgctggcgacgctgacgccgctggcattgggaggctgctcccagccagaggcattaggggggaaggccccgtagtggcaatgcagcgggggcgccagcgtgaagatggggtccgaggccatgcccagagccacgaagagcaccggcaggcagcagaggccgagctgcagctgctggccgccgcccagcgcccccacctgggcgagcagcgcctcaaagctgagggggcctgggggcacggccagcgacaggctgctgcccagtccgtcgccgcccgcgtctccctccccctcccgctcgcgctcccgctcaccctgcagctgctccgtgggcaccgcatctccgagggtcccgactccgttggaggtgggggtgatctctacagtgttgtcgattttgccgccgcccccgccattgggctcgggggtcccggtggccacccggggagccagcttgccgaccgcaggggccctgccggcccgcgccgaaaggatgcgctgtcctctggctcagttgcgcgccggctgcccggacacagacagctcgaagagatcccgctctgcagctctgcagccgcgggcgcctccttggtctctgcgatctctgcgctgctttcccctccccttcctctagactctcctccccttcccacgtcagcagaaccttcggtccagactcttcgtcagagagaggaaggggggccagggcccaggggagggagggaaggggggctctgtcgtctctttcctgggtctgcgggccattgcggtaaaaaagaaaaaaagctgaaggatagtagctagtccaggcagatgccagagattcttcctctgcttccaatcatttgccatcattcattcattcattcattcacccattcactaatcagtaaaatttaagtgtccactacgttccaggacttgcactagactttaaggataacagggtggacaagttccactttggagacctttactccagggagacagacatgtaaactggctattacagtacaacttatgcatatggaagactgtcttggccctgtatcagccctagcttcagtcctctacaaggagaccactttcttgggtttcatcactcccatcctgtttgaatctccatttctcaacagcatttggcactgttgacccctcttcctctaaacactctcttcctttgctgctgagtctctcttgctccccttttctccattgcagaaatcgtcttccagctcatggcattggtgctgagcatgggcaggccattatcctcccggttcttgaggcaatgattgaagtccagcggggtgacgcaactgcaggaggggtctgtattggtagtgatgaggctgtggtgctggcttctagggccattcccgtctgtatcatttagacaccatggttcagtgtctggaatcctcacagacttagtcctaggccctcctctcatctcacactgtctccactttgggatcttacctatgcccacagcttcaatcaccacccatacaaacaatacaaacctgacgcccagactgacatctccagcttccacctctgttctgagctccagacctatgaagccacctcttatttgaccttcaccttggatgactcacagggacctcaaactcaatatgttcaagacgaaatttttgcttttcccccataacttggttggcttccactgcttttttctgcagcgaatggcaccctcaacatcgcattgtggccaaatgctcaggcaacagcctttagagctttctcttccttatccatgttgaattctttacaaaattctgcccattttacttcctatatattctcagacatcccacatctctccatctctaccattattagtcaagctacctgttgcaaagaccactttagctccctaattcctaactggtgttcagcgtccgctttgtttatacctccttatcacccatatgtcatttatagtcagatagaatgatcttttcaaaatacagatctgatcatgtatctttcctgctaaccagccttcagtggtgtctcctcactgtcaaagtgaatattaaaaatctagatacctcatacatggttctacatgcctggtcacatgctgtctgtagttccatctcacttctttccccaaactctctgcactccagccacagaccttcttctagttttcccagcgccacgaggcctttgaacaagctggttcctgcacctaaaaagcttcttagtcacatttttctcatccttcagctctcagcctaaacatctttgctacacaggagtcttccctaacctctagaattgctactcaaagtgtggttcatggaccagcagcattcctgggagcttgttagaaatgcagaatccaagcctcacccagacccttgaatcataatctgtattttatccagatctccaggcataggtattatacattaaaggtagagacacacatctctaagagatttgttacctgataggtactttattctctaatcctaggtaagggctagaaagcagtgttctatcattgtcagccgggaaatctttcccccttctctccactgaaccacacttttaacttgtctctgttcagaaattttccacgtatgggaaactcttttcttcagacagggtctcactgtcttacccaggatggagtgcagtggcttgatcacagctcactgcag

SEQ ID NO: 18919 - RNA, 1555 nt, Homo sapiens
  source 1..1555: mol_type = other RNA
tgcctccttggtctccggcagcagcataatgctgagaatgcagaggagggcgcaggccgccagcaccacgtgctgcaggaaggctccatggcccatgtggaggcgctgggccgggccgctcagtcctccaagcgcccctagagccatgatcaggcccaggccacggccccggacagtggtggggatgacctcagcagcaaggagggtgctgaggatggcggcagcttgggaggagaagagcccaaggacagagaaagtggtgatggcagcctcgttcagataatcccacaggcccagcaggaccagggaagcaatgccggtaagggtcatggagagaagaaggatgccccggcggccaaatcggtccacggtgacccccaggaagacacaggccagggctgcggtgccgctggccagcagagagcacaggtagaagtccgatgggctccctcctcctcccacaggctggtagcagtggcgaatggcatgggcaatgaagttggtgaagcccaggataagcagatttttccagatgttgcggtagttgaggagggaagcaaaggaaaaggaggatgttgcagggagagggcaggtattctccaggtcctgcagggcctcctgggcctcctcccccagcatctgcccatggggccggtttcgctcagccaggatcctcagcacagactgagcctcctcaatctgccgcttcactatcagccaccgtgcggactccaggaacaaaccaggccagccataaaacaggaagaggatgcagggagcggtgatcattcggcatcaggtagacacccaggtcaacaccggcaagcagaaagcccaagaggaatcggagggccatgacgcctgtggaggagcctgcagcagcccctcctactccacaggggcccaccagccccaaggtcagcagcacaatcccgcgacggccaaatctgtctgcggggtaacccaggaacaggtagccggaggcaaagcccaagatgaagaggatctgctccaggatcacctgccagcccaggtcacacaccagatcccactggccgatggcgttggtggtgagcacaggaaggccattatagtcccaatccttgaggcaatggttgaagtccggcggggcgaagccgctgcacgaggggtcggtactggtggcgacacggctggcggcgctggctgctagggcagcgctggcgacgctgacgccgctggcattgggaggctgctcccagccagaggcattaggggggaaggccccgtagtggcaatgcagcgggggcgccagcgtgaagatggggtccgaggccatgcccagagccacgaagagcaccggcaggcagcagaggccgagctgcagctgctggccgccgcccagcgcccccacctgggcgagcagcgcctcaaagctgagggggcctgggggcacggccagcgacaggctgctgcccagtccgtcgccgcccgcgtctccctccccctcccgctcgcgctcccgctcaccctgcagctgctccgtgggcaccgcatctccgagggtcccgacctg

SEQ ID NO: 18920 - RNA, 3702 nt, Homo sapiens
  source 1..3702: mol_type = other RNA
tgcctccttggtctccggcagcagcataatgctgagaatgcagaggagggcgcaggccgccagcaccacgtgctgcaggaaggctccatggcccatgtggaggcgctgggccgggccgctcagtcctccaagcgcccctagagccatgatcaggcccaggccacggccccggacagtggtggggatgacctcagcagcaaggagggtgctgaggatggcggcagcttgggaggagaagagcccaaggacagagaaagtggtgatggcagcctcgttcagatcctgcagggcctcctgggcctcctcccccagcatctgcccatggggccggtttcgctcagccaggatcctcagcacagactgagcctcctcaatctgccgcttcactatcagccaccgtgcggactccaggaacaaaccaggccagccataaaacaggaagaggatgcagggagcggtgatcattcgctgtaggaatcgccaatccttagagacaagggccaggcccaggaacaggaagtgccctcccacccccaccaactcccctgccagggccacccgaagcctctgggttgggtcgcacagctccaggcgcatcaggtagacacccaggtcaacaccggcaagcagaaagcccaagaggaatcggagggccatgacgcctgtggaggagcctgcagcagcccctcctactccacaggggcccaccagccccaaggtcagcagcacaatcccgcgacggccaaatctgtctgcggggtaacccaggaacaggtagccggaggcaaagcccaagatgaagaggatctgctccaggatcacctgccagcccaggtcacacaccagatcccactggccgatggcgttggtggtgagcacaggaaggccattatagtcccaatccttgaggcaatggttgaagtccggcggggcgaagccgctgcacgaggggtcggtactggtggcgacacggctggcggcgctggctgctagggcagcgctggcgacgctgacgccgctggcattgggaggctgctcccagccagaggcattaggggggaaggccccgtagtggcaatgcagcgggggcgccagcgtgaagatggggtccgaggccatgcccagagccacgaagagcaccggcaggcagcagaggccgagctgcagctgctggccgccgcccagcgcccccacctgggcgagcagcgcctcaaagctgagggggcctgggggcacggccagcgacaggctgctgcccagtccgtcgccgcccgcgtctccctccccctcccgctcgcgctcccgctcaccctgcagctgctccgtgggcaccgcatctccgagggtcccgacctgtccgttggaggtgggggtgatctctacagtgttgtcgattttgccgccgcccccgccattgggctcgggggtcccggtggccacccggggagccagcttgccgaccgcaggggccctgccggcccgcgccgaaaggatgcgctgtcctctggctcagttgcgcgccggctgcccggacacagacagctcgaagagatcccgctctgcagctctgcagccgcgggcgcctccttggtctctgcgatctctgcgctgctttcccctccccttcctctagactctcctccccttcccacgtcagcagaaccttcggtccagactcttcgtcagagagaggaaggggggccagggcccaggggagggagggaaggggggctctgtcgtctctttcctgggtctgcgggccattgcggtaaaaaagaaaaaaagctgaaggatagtagctagtccaggcagatgccagagattcttcctctgcttccaatcatttgccatcattcattcattcattcattcacccattcactaatcagtaaaatttaagtgtccactacgttccaggacttgcactagactttaaggataacagggtggacaagttccactttggagacctttactccagggagacagacatgtaaactggctattacagtacaacttatgcatatggaagactgtcttggccctgtatcagccctagcttcagtcctctacaaggagaccactttcttgggtttcatcactcccatcctgtttgaatctccatttctcaacagcatttggcactgttgacccctcttcctctaaacactctcttcctttgctgctgagtctctcttgctccccttttctccattgcagaaatcgtcttccagctcatggcattggtgctgagcatgggcaggccattatcctcccggttcttgaggcaatgattgaagtccagcggggtgacgcaactgcaggaggggtctgtattggtagtgatgaggctgtggtgctggcttctagggccattcccgtctgtatcatttagacaccatggttcagtgtctggaatcctcacagacttagtcctaggccctcctctcatctcacactgtctccactttgggatcttacctatgcccacagcttcaatcaccacccatacaaacaatacaaacctgacgcccagactgacatctccagcttccacctctgttctgagctccagacctatgaagccacctcttatttgaccttcaccttggatgactcacagggacctcaaactcaatatgttcaagacgaaatttttgcttttcccccataacttggttggcttccactgcttttttctgcagcgaatggcaccctcaacatcgcattgtggccaaatgctcaggcaacagcctttagagctttctcttccttatccatgttgaattctttacaaaattctgcccattttacttcctatatattctcagacatcccacatctctccatctctaccattattagtcaagctacctgttgcaaagaccactttagctccctaattcctaactggtgttcagcgtccgctttgtttatacctccttatcacccatatgtcatttatagtcagatagaatgatcttttcaaaatacagatctgatcatgtatctttcctgctaaccagccttcagtggtgtctcctcactgtcaaagtgaatattaaaaatctagatacctcatacatggttctacatgcctggtcacatgctgtctgtagttccatctcacttctttccccaaactctctgcactccagccacagaccttcttctagttttcccagcgccacgaggcctttgaacaagctggttcctgcacctaaaaagcttcttagtcacatttttctcatccttcagctctcagcctaaacatctttgctacacaggagtcttccctaacctctagaattgctactcaaagtgtggttcatggaccagcagcattcctgggagcttgttagaaatgcagaatccaagcctcacccagacccttgaatcataatctgtattttatccagatctccaggcataggtattatacattaaaggtagagacacacatctctaagagatttgttacctgataggtactttattctctaatcctaggtaagggctagaaagcagtgttctatcattgtcagccgggaaatctttcccccttctctccactgaaccacacttttaacttgtctctgttcagaaattttccacgtatgggaaactcttttcttcagacagggtctcactgtcttacccaggatggagtgcagtggcttgatcacagctcactgcagtctc

SEQ ID NO: 18921 - RNA, 3972 nt, Homo sapiens
  source 1..3972: mol_type = other RNA
tgcctccttggtctccggcagcagcataatgctgagaatgcagaggagggcgcaggccgccagcaccacgtgctgcaggaaggctccatggcccatgtggaggcgctgggccgggccgctcagtcctccaagcgcccctagagccatgatcaggcccaggccacggccccggacagtggtggggatgacctcagcagcaaggagggtgctgaggatggcggcagcttgggaggagaagagcccaaggacagagaaagtggtgatggcagcctcgttcagatctctgttggggttcccttgttgagcccacactgtggggaagataggatgctcacaatcccacaggcccagcaggaccagggaagcaatgccggtaagggtcatggagagaagaaggatgccccggcggccaaatcggtccacggtgacccccaggaagacacaggccagggctgcggtgccgctggccagcagagagcacaggtagaagtccgatgggctccctcctcctcccacaggctggtagcagtggcgaatggcatgggcaatgaagcctgcagggcctcctgggcctcctcccccagcatctgcccatggggccggtttcgctcagccaggatcctcagcacagactgagcctcctcaatctgccgcttcactatcagccaccgtgcggactccaggaacaaaccaggccagccataaaacaggaagaggatgcagggagcggtgatcattcgctgtaggaatcgccaatccttagagacaagggccaggcccaggaacaggaagtgccctcccacccccaccaactcccctgccagggccacccgaagcctctgggttgggtcgcacagctccaggcgcatcaggtagacacccaggtcaacaccggcaagcagaaagcccaagaggaatcggagggccatgacgcctgtggaggagcctgcagcagcccctcctactccacaggggcccaccagccccaaggtcagcagcacaatcccgcgacggccaaatctgtctgcggggtaacccaggaacaggtagccggaggcaaagcccaagatgaagaggatctgctccaggatcacctgccagcccaggtcacacaccagatcccactggccgatggcgttggtggtgagcacaggaaggccattatagtcccaatccttgaggcaatggttgaagtccggcggggcgaagccgctgcacgaggggtcggtactggtggcgacacggctggcggcgctggctgctagggcagcgctggcgacgctgacgccgctggcattgggaggctgctcccagccagaggcattaggggggaaggccccgtagtggcaatgcagcgggggcgccagcgtgaagatggggtccgaggccatgcccagagccacgaagagcaccggcaggcagcagaggccgagctgcagctgctggccgccgcccagcgcccccacctgggcgagcagcgcctcaaagctgagggggcctgggggcacggccagcgacaggctgctgcccagtccgtcgccgcccgcgtctccctccccctcccgctcgcgctcccgctcaccctgcagctgctccgtgggcaccgcatctccgagggtcccgacctgtccgttggaggtgggggtgatctctacagtgttgtcgattttgccgccgcccccgccattgggctcgggggtcccggtggccacccggggagccagcttgccgaccgcaggggccctgccggcccgcgccgaaaggatgcgctgtcctctggctcagttgcgcgccggctgcccggacacagacagctcgaagagatcccgctctgcagctctgcagccgcgggcgcctccttggtctctgcgatctctgcgctgctttcccctccccttcctctagactctcctccccttcccacgtcagcagaaccttcggtccagactcttcgtcagagagaggaaggggggccagggcccaggggagggagggaaggggggctctgtcgtctctttcctgggtctgcgggccattgcggtaaaaaagaaaaaaagctgaaggatagtagctagtccaggcagatgccagagattcttcctctgcttccaatcatttgccatcattcattcattcattcattcacccattcactaatcagtaaaatttaagtgtccactacgttccaggacttgcactagactttaaggataacagggtggacaagttccactttggagacctttactccagggagacagacatgtaaactggctattacagtacaacttatgcatatggaagactgtcttggccctgtatcagccctagcttcagtcctctacaaggagaccactttcttgggtttcatcactcccatcctgtttgaatctccatttctcaacagcatttggcactgttgacccctcttcctctaaacactctcttcctttgctgctgagtctctcttgctccccttttctccattgcagaaatcgtcttccagctcatggcattggtgctgagcatgggcaggccattatcctcccggttcttgaggcaatgattgaagtccagcggggtgacgcaactgcaggaggggtctgtattggtagtgatgaggctgtggtgctggcttctagggccattcccgtctgtatcatttagacaccatggttcagtgtctggaatcctcacagacttagtcctaggccctcctctcatctcacactgtctccactttgggatcttacctatgcccacagcttcaatcaccacccatacaaacaatacaaacctgacgcccagactgacatctccagcttccacctctgttctgagctccagacctatgaagccacctcttatttgaccttcaccttggatgactcacagggacctcaaactcaatatgttcaagacgaaatttttgcttttcccccataacttggttggcttccactgcttttttctgcagcgaatggcaccctcaacatcgcattgtggccaaatgctcaggcaacagcctttagagctttctcttccttatccatgttgaattctttacaaaattctgcccattttacttcctatatattctcagacatcccacatctctccatctctaccattattagtcaagctacctgttgcaaagaccactttagctccctaattcctaactggtgttcagcgtccgctttgtttatacctccttatcacccatatgtcatttatagtcagatagaatgatcttttcaaaatacagatctgatcatgtatctttcctgctaaccagccttcagtggtgtctcctcactgtcaaagtgaatattaaaaatctagatacctcatacatggttctacatgcctggtcacatgctgtctgtagttccatctcacttctttccccaaactctctgcactccagccacagaccttcttctagttttcccagcgccacgaggcctttgaacaagctggttcctgcacctaaaaagcttcttagtcacatttttctcatccttcagctctcagcctaaacatctttgctacacaggagtcttccctaacctctagaattgctactcaaagtgtggttcatggaccagcagcattcctgggagcttgttagaaatgcagaatccaagcctcacccagacccttgaatcataatctgtattttatccagatctccaggcataggtattatacattaaaggtagagacacacatctctaagagatttgttacctgataggtactttattctctaatcctaggtaagggctagaaagcagtgttctatcattgtcagccgggaaatctttcccccttctctccactgaaccacacttttaacttgtctctgttcagaaattttccacgtatgggaaactcttttcttcagacagggtctcactgtcttacccaggatggagtgcagtggcttgatcacagctcactgcagtc

SEQ ID NO: 18922 - RNA, 1734 nt, Homo sapiens
  source 1..1734: mol_type = other RNA
tgcctccttggtctccggcagcagcataatgctgagaatgcagaggagggcgcaggccgccagcaccacgtgctgcaggaaggctccatggcccatgtggaggcgctgggccgggccgctcagtcctccaagcgcccctagagccatgatcaggcccaggccacggccccggacagtggtggggatgacctcagcagcaaggagggtgctgaggatggcggcagcttgggaggagaagagcccaaggacagagaaagtggtgatggcagcctcgttcagatctctgttggggttcccttgttgagcccacactgtggggaagataggatgctcacaatcccacaggcccagcaggaccagggaagcaatgccggtaagggtcatggagagaagaaggatgccccggcggccaaatcggtccacggtgacccccaggaagacacaggccagggctgcggtgccgctggccagcagagagcacaggtagaagtccgatgggctccctcctcctcccacaggctggtagcagtggcgaatggcatgggcaatgaagttggtgaagcccaggataagcagatttttccagatgttgcggtagttgaggagggaagcaaaggaaaaggaggatgttgcagggagagggcaggtattctccaggtcctgcagggcctcctgggcctcctcccccagcatctgcccatggggccggtttcgctcagccaggatcctcagcacagactgagcctcctcaatctgccgcttcactatcagccaccgtgcggactccaggaacaaaccaggccagccataaaacaggaagaggatgcagggagcggtgatcattcgctgtaggaatcgccaatccttagagacaagggccaggcccaggaacaggaagtgccctcccacccccaccaactcccctgccagggccacccgaagcctctgggttgggtcgcacagctccaggcgcatcaggtagacacccaggtcaacaccggcaagcagaaagcccaagaggaatcggagggccatgacgcctgtggaggagcctgcagcagcccctcctactccacaggggcccaccagccccaaggtcagcagcacaatcccgcgacggccaaatctgtctgcggggtaacccaggaacaggtagccggaggcaaagcccaagatgaagaggatctgctccaggatcacctgccagcccaggtcacacaccagatcccactggccgatggcgttggtggtgagcacaggaaggccattatagtcccaatccttgaggcaatggttgaagtccggcggggcgaagccgctgcacgaggggtcggtactggtggcgacacggctggcggcgctggctgctagggcagcgctggcgacgctgacgccgctggcattgggaggctgctcccagccagaggcattaggggggaaggccccgtagtggcaatgcagcgggggcgccagcgtgaagatggggtccgaggccatgcccagagccacgaagagcaccggcaggcagcagaggccgagctgcagctgctggccgccgcccagcgcccccacctgggcgagcagcgcctcaaagctgagggggcctgggggcacggccagcgacaggctgctgcccagtccgtcgccgcccgcgtctccctccccctcccgctcgcgctcccgctcaccctgcagctgctccgtgggcaccgcatctccgagggtcccgacctg

SEQ ID NO: 18923 - RNA, 4077 nt, Homo sapiens
  source 1..4077: mol_type = other RNA
tgcctccttggtctccggcagcagcataatgctgagaatgcagaggagggcgcaggccgccagcaccacgtgctgcaggaaggctccatggcccatgtggaggcgctgggccgggccgctcagtcctccaagcgcccctagagccatgatcaggcccaggccacggccccggacagtggtggggatgacctcagcagcaaggagggtgctgaggatggcggcagcttgggaggagaagagcccaaggacagagaaagtggtgatggcagcctcgttcagatctctgttggggttcccttgttgagcccacactgtggggaagataggatgctcacaatcccacaggcccagcaggaccagggaagcaatgccggtaagggtcatggagagaagaaggatgccccggcggccaaatcggtccacggtgacccccaggaagacacaggccagggctgcggtgccgctggccagcagagagcacaggtagaagtccgatgggctccctcctcctcccacaggctggtagcagtggcgaatggcatgggcaatgaagttggtgaagcccaggataagcagatttttccagatgttgcggtagttgaggagggaagcaaaggaaaaggaggatgttgcagggagagggcaggtattctccaggtcctgcagggcctcctgggcctcctcccccagcatctgcccatggggccggtttcgctcagccaggatcctcagcacagactgagcctcctcaatctgccgcttcactatcagccaccgtgcggactccaggaacaaaccaggccagccataaaacaggaagaggatgcagggagcggtgatcattcgctgtaggaatcgccaatccttagagacaagggccaggcccaggaacaggaagtgccctcccacccccaccaactcccctgccagggccacccgaagcctctgggttgggtcgcacagctccaggcgcatcaggtagacacccaggtcaacaccggcaagcagaaagcccaagaggaatcggagggccatgacgcctgtggaggagcctgcagcagcccctcctactccacaggggcccaccagccccaaggtcagcagcacaatcccgcgacggccaaatctgtctgcggggtaacccaggaacaggtagccggaggcaaagcccaagatgaagaggatctgctccaggatcacctgccagcccaggtcacacaccagatcccactggccgatggcgttggtggtgagcacaggaaggccattatagtcccaatccttgaggcaatggttgaagtccggcggggcgaagccgctgcacgaggggtcggtactggtggcgacacggctggcggcgctggctgctagggcagcgctggcgacgctgacgccgctggcattgggaggctgctcccagccagaggcattaggggggaaggccccgtagtggcaatgcagcgggggcgccagcgtgaagatggggtccgaggccatgcccagagccacgaagagcaccggcaggcagcagaggccgagctgcagctgctggccgccgcccagcgcccccacctgggcgagcagcgcctcaaagctgagggggcctgggggcacggccagcgacaggctgctgcccagtccgtcgccgcccgcgtctccctccccctcccgctcgcgctcccgctcaccctgcagctgctccgtgggcaccgcatctccgagggtcccgacctgtccgttggaggtgggggtgatctctacagtgttgtcgattttgccgccgcccccgccattgggctcgggggtcccggtggccacccggggagccagcttgccgaccgcaggggccctgccggcccgcgccgaaaggatgcgctgtcctctggctcagttgcgcgccggctgcccggacacagacagctcgaagagatcccgctctgcagctctgcagccgcgggcgcctccttggtctctgcgatctctgcgctgctttcccctccccttcctctagactctcctccccttcccacgtcagcagaaccttcggtccagactcttcgtcagagagaggaaggggggccagggcccaggggagggagggaaggggggctctgtcgtctctttcctgggtctgcgggccattgcggtaaaaaagaaaaaaagctgaaggatagtagctagtccaggcagatgccagagattcttcctctgcttccaatcatttgccatcattcattcattcattcattcacccattcactaatcagtaaaatttaagtgtccactacgttccaggacttgcactagactttaaggataacagggtggacaagttccactttggagacctttactccagggagacagacatgtaaactggctattacagtacaacttatgcatatggaagactgtcttggccctgtatcagccctagcttcagtcctctacaaggagaccactttcttgggtttcatcactcccatcctgtttgaatctccatttctcaacagcatttggcactgttgacccctcttcctctaaacactctcttcctttgctgctgagtctctcttgctccccttttctccattgcagaaatcgtcttccagctcatggcattggtgctgagcatgggcaggccattatcctcccggttcttgaggcaatgattgaagtccagcggggtgacgcaactgcaggaggggtctgtattggtagtgatgaggctgtggtgctggcttctagggccattcccgtctgtatcatttagacaccatggttcagtgtctggaatcctcacagacttagtcctaggccctcctctcatctcacactgtctccactttgggatcttacctatgcccacagcttcaatcaccacccatacaaacaatacaaacctgacgcccagactgacatctccagcttccacctctgttctgagctccagacctatgaagccacctcttatttgaccttcaccttggatgactcacagggacctcaaactcaatatgttcaagacgaaatttttgcttttcccccataacttggttggcttccactgcttttttctgcagcgaatggcaccctcaacatcgcattgtggccaaatgctcaggcaacagcctttagagctttctcttccttatccatgttgaattctttacaaaattctgcccattttacttcctatatattctcagacatcccacatctctccatctctaccattattagtcaagctacctgttgcaaagaccactttagctccctaattcctaactggtgttcagcgtccgctttgtttatacctccttatcacccatatgtcatttatagtcagatagaatgatcttttcaaaatacagatctgatcatgtatctttcctgctaaccagccttcagtggtgtctcctcactgtcaaagtgaatattaaaaatctagatacctcatacatggttctacatgcctggtcacatgctgtctgtagttccatctcacttctttccccaaactctctgcactccagccacagaccttcttctagttttcccagcgccacgaggcctttgaacaagctggttcctgcacctaaaaagcttcttagtcacatttttctcatccttcagctctcagcctaaacatctttgctacacaggagtcttccctaacctctagaattgctactcaaagtgtggttcatggaccagcagcattcctgggagcttgttagaaatgcagaatccaagcctcacccagacccttgaatcataatctgtattttatccagatctccaggcataggtattatacattaaaggtagagacacacatctctaagagatttgttacctgataggtactttattctctaatcctaggtaagggctagaaagcagtgttctatcattgtcagccgggaaatctttcccccttctctccactgaaccacacttttaacttgtctctgttcagaaattttccacgtatgggaaactcttttcttcagacagggtctcactgtcttacccaggatggagtgcagtggcttgatcacagctcactgcagt

SEQ ID NO: 18924 - RNA, 4074 nt, Homo sapiens
  source 1..4074: mol_type = other RNA
tgcctccttggtctccggcagcagcataatgctgagaatgcagaggagggcgcaggccgccagcaccacgtgctgcaggaaggctccatggcccatgtggaggcgctgggccgggccgctcagtcctccaagcgcccctagagccatgatcaggcccaggccacggccccggacagtggtggggatgacctcagcagcaaggagggtgctgaggatggcggcagcttgggaggagaagagcccaaggacagagaaagtggtgatggcagcctcgttcagatctctgttggggttcccttgttgagcccacactgtggggaagataggatgctcacaatcccacaggcccagcaggaccagggaagcaatgccggtaagggtcatggagagaagaaggatgccccggcggccaaatcggtccacggtgacccccaggaagacacaggccagggctgcggtgccgctggccagcagagagcacaggtagaagtccgatgggctccctcctcctcccacaggctggtagcagtggcgaatggcatgggcaatgaagttggtgaagcccaggataagcagatttttccagatgttgcggtagttgaggagggaagcaaaggaaaaggaggatgttgcagggagagggcaggtattctccaggtcctgcagggcctcctgggcctcctcccccagcatctgcccatggggccggtttcgctcagccaggatcctcagcacagactgagcctcctcaatctgccgcttcactatcagccaccgtgcggactccaggaacaaaccaggccagccataaaacaggaagaggatgcagggagcggtgatcattcgctgtaggaatcgccaatccttagagacaagggccaggcccaggaacaggaagtgccctcccacccccaccaactcccctgccagggccacccgaagcctctgggttgggtcgcacagctccaggcgcatcaggtagacacccaggtcaacaccggcaagcagaaagcccaagaggaatcggagggccatgacgcctgtggaggagcctgcagcagcccctcctactccacaggggcccaccagccccaaggtcagcagcacaatcccgcgacggccaaatctgtctgcggggtaacccaggaacaggtagccggaggcaaagcccaagatgaagaggatctgctccaggatcacctgccagcccaggtcacacaccagatcccactggccgatggcgttggtggtgagcacaggaaggccattatagtcccaatccttgaggcaatggttgaagtccggcggggcgaagccgctgcacgaggggtcggtactggtggcgacacggctggcggcgctggctgctagggcagcgctggcgacgctgacgccgctggcattgggaggctgctcccagccagaggcattaggggggaaggccccgtagtggcaatgcagcgggggcgccagcgtgaagatggggtccgaggccatgcccagagccacgaagagcaccggcaggcagcagaggccgagctgcagctgctggccgccgcccagcgcccccacctgggcgagcagcgcctcaaagctgagggggcctgggggcacggccagcgacaggctgctgcccagtccgtcgccgcccgcgtctccctccccctcccgctcgcgctcccgctcaccctgcagctgctccgtgggcaccgcatctccgagggtcccgactccgttggaggtgggggtgatctctacagtgttgtcgattttgccgccgcccccgccattgggctcgggggtcccggtggccacccggggagccagcttgccgaccgcaggggccctgccggcccgcgccgaaaggatgcgctgtcctctggctcagttgcgcgccggctgcccggacacagacagctcgaagagatcccgctctgcagctctgcagccgcgggcgcctccttggtctctgcgatctctgcgctgctttcccctccccttcctctagactctcctccccttcccacgtcagcagaaccttcggtccagactcttcgtcagagagaggaaggggggccagggcccaggggagggagggaaggggggctctgtcgtctctttcctgggtctgcgggccattgcggtaaaaaagaaaaaaagctgaaggatagtagctagtccaggcagatgccagagattcttcctctgcttccaatcatttgccatcattcattcattcattcattcacccattcactaatcagtaaaatttaagtgtccactacgttccaggacttgcactagactttaaggataacagggtggacaagttccactttggagacctttactccagggagacagacatgtaaactggctattacagtacaacttatgcatatggaagactgtcttggccctgtatcagccctagcttcagtcctctacaaggagaccactttcttgggtttcatcactcccatcctgtttgaatctccatttctcaacagcatttggcactgttgacccctcttcctctaaacactctcttcctttgctgctgagtctctcttgctccccttttctccattgcagaaatcgtcttccagctcatggcattggtgctgagcatgggcaggccattatcctcccggttcttgaggcaatgattgaagtccagcggggtgacgcaactgcaggaggggtctgtattggtagtgatgaggctgtggtgctggcttctagggccattcccgtctgtatcatttagacaccatggttcagtgtctggaatcctcacagacttagtcctaggccctcctctcatctcacactgtctccactttgggatcttacctatgcccacagcttcaatcaccacccatacaaacaatacaaacctgacgcccagactgacatctccagcttccacctctgttctgagctccagacctatgaagccacctcttatttgaccttcaccttggatgactcacagggacctcaaactcaatatgttcaagacgaaatttttgcttttcccccataacttggttggcttccactgcttttttctgcagcgaatggcaccctcaacatcgcattgtggccaaatgctcaggcaacagcctttagagctttctcttccttatccatgttgaattctttacaaaattctgcccattttacttcctatatattctcagacatcccacatctctccatctctaccattattagtcaagctacctgttgcaaagaccactttagctccctaattcctaactggtgttcagcgtccgctttgtttatacctccttatcacccatatgtcatttatagtcagatagaatgatcttttcaaaatacagatctgatcatgtatctttcctgctaaccagccttcagtggtgtctcctcactgtcaaagtgaatattaaaaatctagatacctcatacatggttctacatgcctggtcacatgctgtctgtagttccatctcacttctttccccaaactctctgcactccagccacagaccttcttctagttttcccagcgccacgaggcctttgaacaagctggttcctgcacctaaaaagcttcttagtcacatttttctcatccttcagctctcagcctaaacatctttgctacacaggagtcttccctaacctctagaattgctactcaaagtgtggttcatggaccagcagcattcctgggagcttgttagaaatgcagaatccaagcctcacccagacccttgaatcataatctgtattttatccagatctccaggcataggtattatacattaaaggtagagacacacatctctaagagatttgttacctgataggtactttattctctaatcctaggtaagggctagaaagcagtgttctatcattgtcagccgggaaatctttcccccttctctccactgaaccacacttttaacttgtctctgttcagaaattttccacgtatgggaaactcttttcttcagacagggtctcactgtcttacccaggatggagtgcagtggcttgatcacagctcactgcagt

SEQ ID NO: 18925 - RNA, 319 nt, Homo sapiens
  source 1..319: mol_type = other RNA
tgcctccttggtctccggcaggctggtccagagcctggcccccagcccctgaagcagggccgggggactgcgtgctacataggtggggctgatccctctcacattgaggctcgggtgtatcagaggacatgtgacttcaatttacatgaattgttctctgcaatctccatgacaacccataaggcaagtacataatcatccccaacctacagatgaggaaatagaggctctggcctcagtttacatactctctgaagatgtattttcttttttttcttttttttttttttttgagatggagtttcgctcttgttgccca

SEQ ID NO: 18926 - RNA, 27 nt, Homo sapiens
  source 1..27: mol_type = other RNA
tgcctggaacatagtagggactcaata

SEQ ID NO: 18927 - RNA, 30 nt, Homo sapiens
  source 1..30: mol_type = other RNA
tgcctggaacatagtagggactcaataaag

SEQ ID NO: 18928 - RNA, 71 nt, Homo sapiens
  source 1..71: mol_type = other RNA
tgcctgtctacacttgctgtgcagaacatccgctcacctgtacagcaggcacagacaggcagtcacatgac

SEQ ID NO: 18929 - RNA, 7857 nt, Homo sapiens
  source 1..7857: mol_type = other RNA
tgcctgtctacacttgctgtgcagaacatccgctcacctgtacagcaggcacagacaggcagtcacatgacaacccagcctgaatgacaaccagccattgaaagaaagcagccctcacaccatagcatctacaccaagagctacaaccaaaatgaggggctcgggggcctggggttttaatctgttggtttaatacttaactcatgtattattttattttgattcaagtattaaaacccaccaaaagtaaagtgagtggtgcctatgaaatataataaaacccatttctgaaaatgttcctgtgcattctatagttctcttttcctaattgttgtcagcaaatcactacccttgacctttattgtacacagctttgcagcaccctatattgatataaaaactcaatataacaaaacaatataacttcagtctgatgcttaacaaagaataaattattctaagaattcttgtccataaactaagtatggttttctatgtcatgattttttttttttttttttttttttggaaggggatagggtggaaagacagagaaaagaaaagggagaaaaagagtattccaaaggatcaagtgctttgagttaactctgccagtctgggttaactctgccagtctgggtctgggcaaaacacagtgaaaagactactatttccaactagtgttcaactatattaaaataatagtttctcctcttttgacatatggaaagttgaaatttttgatacttccacgcgtcatggtatacataaatttatgactgcgtcattctttaattaagaaggtgcttatgctacagttctaggagtagaatttacaaggccaacacattcacttgcaacctatgcttccatcactataaactttcaagatcttgagatgttcaggcaattcatttatcttcagaagcataaggaaagtggttaatgcacttgaaatgtatattttgacacatcttttgagaaaatatccaaacttcagtttatgcactgttaactggagtgaaatgataagggatggcttttgtctatgaatactttaaatacttaagggtaaaaggtgggaagatggataaaattagaaatgtgtcaacttttatttagttcattaacatgttttagcttcagtatttgaaattaattttcatctttcttagattctggtcaagcttaaaaaatgtaacacaaggctactcaaaacttttttcacatttaacaattaaacactttatgtatgtattcttaactaaagcaaactatttttcattcagctattttatttttaaaatgaaagtctcagtcttaaagctaagatcccagtgagtttcaaattttctgacaatgatattttaaccaaacctgacattatagtttctttaattaaaaaactgaatgatggggcaaaactacaaagcacaaatatgattaaagttaaatttctctcatttaaacaatcttgtcttatggcaatatgtcatctgctaaaattcatctctgcttctgcaagatacattgcacgatgcagatttttgccttaaataaaagtcccattactagcaaataaagtcctaaacaatacttacaaaatgtagaatataaacaggaagacaatataaaaattactcacagaatatcgacatcgttctacccaatcttaaatgccttgtaccacctgttgcaaatgctgcctatgagagttcacgtatggaattattctactggaccctgcaaggctcaggagagtgcttgacagctcccagaatgagacaatgacctagccagaacattaaggagactacacccgtccttcagactccaaagggaaagctaggacggcagcagagtcatcctaaggtgaggcactccaggataacattttcaatatttttccttaaaacataaagttaacaccttttttgttaaacattttttactcaattttcaaaaaaaatgcttgaaagaatgttttgtatgtattttaaagtcattaaatgaggcacatttaaaaatttttctcttctgggaaagggtaatataaaggataatattgctcttccaggataaacttttgagtgggacaaataatgcatataggggagtgggtttgaatctaaactcatttttaataaatttggaataggattggccattatggtttattgaataatactctttttttcaaaattataaatctttagataataccagaacatggaaatatttgtatgaataatcctatattaaaaaagaataacatcagatagtttatgtatgtaaaaaaatatacaactgtgatcatgcagaattttaagtaatataagtggattagagttcaatatttactgggacttttgtgaaaatatctaagttttggctaactaaataacttaacgaaggagtgtgaacagtgttcacagggtcgacgctgaccttttccaccacagggagtgtgcagatctggtaggaaatatgcacaatcttaaaagtataagtgaaactagaaagagagctgaatatttctataacttcttgatctcacaactttgatcatccagggatataactgtcattttgtttcctatttctgaagttacatttgtcatttgttattgttacaaaatgaaaacaatgctaagtaaatatccctataagggaattatataatctccttatcaagttatccaaacacttcaacccacaaaaatgaggcctgtaatttcttaagagtccaaagaatgtccttatttcaatgcagatgttgggttttcctcaatagtataaggttagcagatttccactggaaacgcctatgttgcattattctgcttgcctaggagtagctcattatgatttaaatctttacacactgggctatagaaatagaataaatattgactaagtgcttttattatacataaattaacagtcctctttcttcagagatttgaattatctcttaaaatttacatatttatgtatttttaaaacaaatttctcattggttttaagaaaaataaggctcttttctccttgaatcagggtctcccattctcctaaaattcacattttagacataagttaaagaaaagccatcatttttttcaagtctgattttaaagtattaatgtaaaattatctagatcaaaaatccatttcaaaaaacttttgaaatgacagtttctgttttattctcacatcttgctttttactaaatccctttccaaaaatgtacaacatatatgggcaatgtatgaaaacaacattgggaaattaattttctgtttaaatgattttcaatccaggaagtcacatatatatagtcagaggataaaaaacaaacaaacaaacaaaaaacaaaaacaaaaacaaaaaaacactaaccttcaatgatgaaaattaacaaaatttaagacaatttaagacaatctacctttagtggtaattttattctgtaattcaataatttaattttgacacttgatatgccaggacgtgattaattattatgctgcatttattcattcatttgctcaatgacaccttcattcaatcaatatttagttagtgtctcctatcagtgctatgtcccctggtggtaggacagggaacaaacaatgtctcctggtctcaagaggcttacagtttgctgcaactcttagcatgtgtgatgagttgttcatgtcaattttcaccttccaaaaacatctcttaaatccgttcatttttatcaaattccaacaactcatcccagcccaagctaccattatctatgcagaccacaatagatgtagaaagcaatagctttctagtaactccccagtccagtttcgccctcttccaatccattctccacaaggcaaccaaaggaatcagtaaagaattcaaatcttatcatgtgactctccagcttaaaaaacttctcatcattcttaatatcaaaatcctcatctttagagtgcctttctctttttgctccagtcacactggacttaattaccctccttaaattcatcaggctcaatcctgcctcagaacattaacacaaaccttctctgaccatccaatgtaaagtaccccctacctgtgtcctctatcccagacactctatgtcaactcatcactggctttattttcttcctagcctgtaatcagcatctgctaggttttcctatttatttgtatgtttgctttattgggaaagagccttcataagaataggtaccatgaattccttgctaatcattttatccttagtgattaggacagtgcctggtacataacaagtgttcagaaagtaattgttgggaaatgttcagatgattaagagcacagcactgacacttagcacctggctaagttactcactctcttttgagcctcaattctttatctctaaaatggagaatgtaaataatgtgctcagtgaactataaatactcaataactattagccattatggtgatgatcctcctcattaagatcatcattgagtttgagttgtggttgcaagtagcattccccctagtcattatacctgcttaaattcacgaaggccagctttcagtctcaatgatgatcttaatgatgagaacttcctgtcttgtttcttgagagttctgaatgagtaacagaagctagtgactcaatcatagctgtgtgtagcccataattttgctaccttgaacttaagtgctccgcaccctcaccaccagctactacccagccaccatcctctcttgcctggaccatggtcagagtttccaatctggtctcccttcttccatgctagccatccccgctcccttcacgcatccaccccataccacttattatgcacaatccagcagccagggcaatctttctaaaccatcaatccaatcatgtcacaacctgttggaacactccaatcattttcagttatccttgtaataaaatccaaaccattgggtagggactgataaggcccccatctactggtacctctgattttatctcctttctcccccactgttcctatgttacagccacagacttcctgttggatcccatctccagggtttttatacttactgttccctctacctggaatattcttcagcaaaatcttctgcacagctcatcatctcagtctctgctcaagtggtacttccttccaatcacccaaatctaaagacccctcccctatcactttctaactcaatgccccattttattttcttcagagcatttactatctgacatttattactagtctatttgcttgttagctccatagaacagtaactttgtcatttcctcttttttaaaatgatctaaatggatgaaactaccctttcctagaatttcttcatctaaataattccatttatttcaagggtcatttccactctcacctgcccccaactaccctccataccataccttggttatacacagcacacagagcgggagtattcatggcacttggttaatattataactgtgcatatttattttccatttgttgtaatcaagtactcataaggaagctacaagggcagtgattttgtaaagaattatcctgagtctggaggagaggagatgagccaataaccaagagctcaccaagccttcaaagcttcttccttccctacagagagcatcctataccttccaatgggcttattttcaggactcacagagccagactaatgccacactccaacagcagtagctactccagagtcttcagtgtctctgctgctaacacccaggaacatgtcaatgctgagatgcctggaattcatcttcataagtcctctgtgggatgaggttggcttggacaactccaggcatctctgggattcttgcctttatttgtggttgaaagcataggctctggagctcaacagcctgggttcaaatttctgctttgccaccaactagctgtgtgactttggtaagttggttatcctcgccaagactaaatgttctcatcatctttataccaggacaagctttccgcagtaaggacgaaccagtatcccttcgagccgcctttcatgatgccaatgttgctgatggtgagccaccccttgcgaatcacagaacttagctcgtacaatttgccttgaaggcggaagattggttccctgatttccaactgtggttttcttgtgaacctgactgctcctctgctgagcatttgcgaagccaatgaagtcttcatggttggtgttgatgtaagagacttgaatgtcaatcaatagcaatacctggtcctttgtcttcccttctcgctcacgaatgtggttagcaacaatcctttccgtttcctcgcagagtctggggaagtttgccagttttttggtacacttcttcacagtgttgattaattcttgtattaccagatccacactcttcaaggaaggccctttcaactttacaatctgtttcttgactatcgcttcaaatgccatgtctggagtaaacaaccctgtcctgataccatgtatgtttttgattgcatagcttatttctcttcgcaattctttctcattgaactccatctttactatctcaaaaggaaagcgttcatgaaaaatacgattgattttagcaccacctgagagttccagggtatctacttgatcccctgacccttcaattctcttctcaaagtccacagcaaattgctgaaccatctgcagcaatgctttggtcttccttgttgggtcttctggtttgaaatttttgtaggcttctacttcatgttctatggagagcaactgtccctgtagtttgttcctgaagtttggtagggtatcccgaatgtggttggtaagttgctgattaaggaccttctgcaggtgtggggttcccattcggtcagcgatatgtctgtaagccgggtgggaaaggaaaaacttcctctctgccagcatggctgcctttatgtccttcttcccatctatgtccttctggcttctgtttaccacccccacgtaacccctgcgaagaggcaacagtttgttctctagaacatccctggcatccgttccttcatccataaggtccagtttggtgataactccaatggttctcagaccttgaggatcaacttctttagctagcttcagcgcatctgagtttgcaagatcagtgttggctggagtaacagctaaaatcagacagttctccctcgtgatgaactgcataatcatttctctgatctgatactcgatatctggtggctgatctcccacaggcactttagttattccaggtagatcaataagggttagatttaacacgtgtggggaatagactcgtaaattaatgggtatggaggaaatgcctttattcattccagtcacgcgatctgtttctgcttcaatctcaaggcgaacttcatcaaaatctgtaaatttctttcctttgcaatgtagaaactcggcatattctgctttagaagtaacaagctgcagcacaagaggtcgtcttgttacaatgcccgaccctcgagggagaaagtccctgcccacgaagttctcgagcaccgagctcttgccggcgctctggccgcccaccacggcgatctgcggcagctccagcaggcagctctgtcccagcgccgaaaacgcgtcctgcagacggttcaccagcgggatcagctcctccatctcccggttccccatcttgcccgaggggccggcgaccagctggtccctgctcgcctctacgacctgacagggagtaggggccgcgctgccctggctgctgctgctgcgccgggctcagccagccaggtcctggcgcagacgtcggagcccgccgccagcccgccgcttggctctgac

SEQ ID NO: 18930 - RNA, 1577 nt, Homo sapiens
  source 1..1577: mol_type = other RNA
tgcggggacaggccagggcatcaggccaggcgcgctcggtgcacaccgcacctgggaggacctgggtacactcaggagaccaagagcactggcgggtcaggatggttggcgttcagctcctacggggtggggagaagtctgtagccgagagcccagccccctcctgccaggtcttcccaggttcgagagaggctggaactcaatttctgcagaaaatctcccagtttttcctgtttggttagtttttttacaaagacaggatcttgctgtgttgcccaggctggtcttgaactcctggcctcaagcaatcctcccacctcggcctccgaaagtgctgggattactggcatgaaccactgcgcccggctggagctcccggtttttaagcactgcacgatactagaagagctgaccttttttctggcctcacagcttatgctgaagctgagtgtgaggaacagagagacctttctgtgacgaccgctggggcagagtggtctatgcgccgagatcctggcatcagcaagggaggcgggtcctcggggaggggcagcttccacagtgtggctgcagcgtgcacagccaggtaggccctggatgttcacccctcactgcccttggggaagcacctgaccgctggggatgtccaccagggagaggacgctgtgtcggggacaacatgcagcatcagcacccacaagggcccggcctggccccgcctctccactcgcccgaggtcttgctgtggcccaaagcaggagtccagggctggcgagacctccggctgcagaaaggcaggcccaggcctcacgatggagaaagtctggatgtcctggtctggcctgctgtttcatgcagtgtgcaagcagcagcatgagcaggcaataggccaactcggctggaggcaccaactgaagccaaggccacgggtcctgtgggcggtgcacgggctcaggcacaccgggaatgtgccacgggtcctgtgggcggtgcacgggctcaggcacaccgggaatgtgccacgggtcctgtgggcggtgcacgggctcaggcacaccgggaatgtgccacgggtcctgtgggcggtgcacgggctcaggcacaccgggaatgtgccatgggtcctgtgggcggtgcacgggctcaggcacagtggggctgtcagctctggcttgcagggtcaccggcctcactgtcgctgctctgagacagctctgtggggctctcaaggcagtgcagctccaggaagctggtgatgagcttggcgatggcttccacatcactgcggtggcccatgactgcactctgcgtgagggggtgggagaagcccgtcgcaagccggagcaccaccatgtagcctttcccgaagtaccggaccttctcctcctccacgctcacatcacggacatcatggagcaggaccaccacctggtcgtggccagctctgaaaagagtcagcagcttcttgtagaggctgaacgtcttcaaaacaaccttccctgtgctcttgtcgaagatggcttccgagagcacagcggtccccgcgccgcagcagagagacgcgaaccggcgggggc

SEQ ID NO: 18931 - RNA, 1774 nt, Homo sapiens
  source 1..1774: mol_type = other RNA
tgcggggacaggccagggcatcaggccaggcgcgctcggtgcacaccgcacctgggaggacctgggtacactcaggagaccaagagcactggcgggtcaggatggttggcgttcagctcctacggggtggggagaagtctgtagccgagagcccagccccctcctgccaggtcttcccaggttcgagagaggctggaactcaatttctgcagaaaatctcccagtttttcctgtttggttagtttttttacaaagacaggatcttgctgtgttgcccaggctggtcttgaactcctggcctcaagcaatcctcccacctcggcctccgaaagtgctgggattactggcatgaaccactgcgcccggctggagctcccggtttttaagcactgcacgatactagaagagctgaccttttttctggcctcacagcttatgctgaagctgagtgtgaggaacagagagacctttctgtgacgaccgctggggcagagtggtctatgcgccgagatcctggcatcagcaagggaggcgggtcctcggggaggggcagcttccacagtgtggctgcagcgtgcacagccaggtaggccctggatgttcacccctcactgcccttggggaagcacctgaccgctggggatgtccaccagggagaggacgctgtgtcggggacaacatgcagcatcagcacccacaagggcccggcctggccccgcctctccactcgcccgaggtcttgctgtggcccaaagcaggagtccagggctggcgagacctccggctgcagaaaggcaggcccaggcctcacgatggagaaagtctggatgtcctggtctggcctgctgtttcatgcagtgtgcaagcagcagcatgagcaggcaataggccaactcggctggaggcaccaactgaagccaaggccacgggtcctgtgggcggtgcacgggctcaggcacaccgggaatgtgccacgggtcctgtgggcggtgcacgggctcaggcacaccgggaatgtgccacgggtcctgtgggcggtgcacgggctcaggcacaccgggaatgtgccacgggtcctgtgggcggtgcacgggctcaggcacaccgggaatgtgccatgggtcctgtgggcggtgcacgggctcaggcacagtggggctgtcagctctggcttgcagggtcaccggcctcactgtcgctgctctgagacagctctgtggggctctcaaggcagtgcagctccaggaagctggtgatgagcttggcgatggcttccacatcactgcggtggcccatgactgcactctgcgtgagggggtgggagaagcccgtcgcaagccggagcaccaccatgtagcctttcccgaagtaccggaccttctcctcctccacgctcacatcacggacatcatggagcaggaccaccacctggtcgtggccagctctgaaaagagtcagcagcttcttgtagaggctgaacgtcttcaaaacaaccttccctgtgctcttgtcgaagatggcttcctcccagtcctccaagttctgcacagccacaaacaggcagcctgtgacgtagaagagcttccagcccaggctatcaaccagcagggaccaggaccggatgcctggagccctcttcagatggaggcgggagctggtgcgggtctccacctgcaggtacatcccgagagggcagcaccactctctacaggaggaggggtcgagagcacagcggtccccgcgccgcagcagagagacgcgaaccggcgggggc

SEQ ID NO: 18932 - RNA, 2902 nt, Homo sapiens
  source 1..2902: mol_type = other RNA
tgcggggacaggccagggcatcaggccaggcgcgctcggtgcacaccgcacctgggaggacctgggtacactcaggagaccaagagcactggcgggtcaggatggttggcgttcagctcctacggggtggggagaagtctgtagccgagagcccagccccctcctgccaggtcttcccaggttcgagagaggctggaactcaatttctgcagaaaatctcccagtttttcctgtttggttagtttttttacaaagacaggatcttgctgtgttgcccaggctggtcttgaactcctggcctcaagcaatcctcccacctcggcctccgaaagtgctgggattactggcatgaaccactgcgcccggctggagctcccggtttttaagcactgcacgatactagaagagctgaccttttttctggcctcacagcttatgctgaagctgagtgtgaggaacagagagacctttctgtgacgaccgctggggcagagtggtctatgcgccgagatcctggcatcagcaagggaggcgggtcctcggggaggggcagcttccacagtgtggctgcagcgtgcacagccaggtaggccctggatgttcacccctcactgcccttggggaagcacctgaccgctggggatgtccaccagggagaggacgctgtgtcggggacaacatgcagcatcagcacccacaagggcccggcctggccccgcctctccactcgcccgaggtcttgctgtggcccaaagcaggagtccagggctggcgagacctccggctgcagaaaggcaggcccaggcctcacgatggagaaagtctggatgtcctggtctggcctgctgtttcatgcagtgtgcaagcagcagcatgagcaggcaataggccaactcggctggaggcaccaactgaagccaaggccacgggtcctgtgggcggtgcacgggctcaggcacaccgggaatgtgccacgggtcctgtgggcggtgcacgggctcaggcacaccgggaatgtgccacgggtcctgtgggcggtgcacgggctcaggcacaccgggaatgtgccacgggtcctgtgggcggtgcacgggctcaggcacaccgggaatgtgccatgggtcctgtgggcggtgcacgggctcaggcacagtggggctgtcagctctggcttgcagggtcaccggcctcactgtcgctgctctgagacagctctgtggggctctcaaggcagtgcagctccaggaagctggtgatgagcttggcgatggcttccacatcactgcggtggcccatgactgcactctgcgtgagggggtgggagaagcccgtcgcaagccggagcaccaccatgtagcctttcccgaagtaccggaccttctcctcctccacgctcacatcacggacatcatggagcaggaccaccacctggtcgtggccagctctgaaaagagtcagcagcttcttgtagaggctgaacgtcttcaaaacaaccttccctgtgctcttgtcgaagatggcttcctcccagtcctccaagttctgcacagccacaaacaggcagcctgtgacgtagaagagcttccagcccaggctatcaaccagcagggaccaggaccggatgcctggagccctcttcagatggaggcgggagctggtgcgggtctccacctgcaggtacatcccgagagggcagcaccactctctacaggaggaggggtctgggaacagacagaggcagctgagcccttgggcctgcacacaggcaggcgcccacgccatcaggcccagtctggaggccaagagcaggtcccccaactaagtcacctgcagccccagacaccatcagccagtctcacctggtctctgtggttgggcacgtcactggatcccccagagaccccgtttcctgtgtaaggaaggcccttttccgttcacagcgacaccgactgcgcgggggctgtttcccgctcagactcacgagctacagctgcatcaccacctgccccgtcctgtctggaaaccttatgtcctgaggccgctagcccccagcagcctttaagcttctagcatctgtgggcaccccctctcccctgtgctggcctccaccaagaaaggaactgaaagtcccatcatggcttccggccgtactggctctcgcactggcatggaccaacgatctcagctctctctctgccctcctccacctgctgaaagttcagactgcacagtagagggtcccaaagcggccagaaccgacgagtcaccaaaggggctaatcttccacagcggagttccgcacgggcgcagcagccctgccacttcaccgtacgctcccaacactggccccagggaccccgttctggtagtttctcagggctttccctgtgaagtcaaatcaaatttctgacattaagtagggggttcaggctgggcgcggtggctcaggcctgtaatctcagcactttgggaggacgaggcgtgcggattgtttgagtcacggagttcaagaccagccagggcaacgtggcgaaaccccgtctccacagaaaatacataaaacagcccggtgtggtggtgtacgcctgtggtcctagttattcaggaggctgagctgggaggatcacctgaggccgggaggtggaggctgcagtgagcagaaatcgtgccactggactccagcctgggtgacagagtgagaccgtgtctcaaaaaaataaaaaatagtgggttcaaatcacacaaaccaatcctagatgctggtatatgactgggctccctcccgggcctcagttgcctcattgctcccgaaacacccggcattccacatccaaatgcacacacacacgcacactcgcggacacaagcacacgcgcgctggcaaagccgcccgcgccgctag

SEQ ID NO: 18933 - RNA, 1896 nt, Homo sapiens
  source 1..1896: mol_type = other RNA
tgcggggacaggccagggcatcaggccaggcgcgctcggtgcacaccgcacctgggaggacctgggtacactcaggagaccaagagcactggcgggtcaggatggttggcgttcagctcctacggggtggggagaagtctgtagccgagagcccagccccctcctgccaggtcttcccaggttcgagagaggctggaactcaatttctgcagaaaatctcccagtttttcctgtttggttagtttttttacaaagacaggatcttgctgtgttgcccaggctggtcttgaactcctggcctcaagcaatcctcccacctcggcctccgaaagtgctgggattactggcatgaaccactgcgcccggctggagctcccggtttttaagcactgcacgatactagaagagctgaccttttttctggcctcacagcttatgctgaagctgagtgtgaggaacagagagacctttctgtgacgaccgctggggcagagtggtctatgcgccgagatcctggcatcagcaagggaggcgggtcctcggggaggggcagcttccacagtgtggctgcagcgtgcacagccaggtaggccctggatgttcacccctcactgcccttggggaagcacctgaccgctggggatgtccaccagggagaggacgctgtgtcggggacaacatgcagcatcagcacccacaagggcccggcctggccccgcctctccactcgcccgaggtcttgctgtggcccaaagcaggagtccagggctggcgagacctccggctgcagaaaggcaggcccaggcctcacgatggagaaagtctggatgtcctggtctggcctgctgtttcatgcagtgtgcaagcagcagcatgagcaggcaataggccaactcggctggaggcaccaactgaagccaaggccacgggtcctgtgggcggtgcacgggctcaggcacaccgggaatgtgccacgggtcctgtgggcggtgcacgggctcaggcacaccgggaatgtgccacgggtcctgtgggcggtgcacgggctcaggcacaccgggaatgtgccacgggtcctgtgggcggtgcacgggctcaggcacaccgggaatgtgccatgggtcctgtgggcggtgcacgggctcaggcacagtggggctgtcagctctggcttgcagggtcaccggcctcactgtcgctgctctgagacagctctgtggggctctcaaggcagtgcagctccaggaagctggtgatgagcttggcgatggcttccacatcactgcggtggcccatgactgcactctgcgtgagggggtgggagaagcccgtcgcaagccggagcaccaccatgtagcctttcccgaagtaccggaccttctcctcctccacgctcacatcacggacatcatggagcaggaccaccacctggtcgtggccagctctgaaaagagtcagcagcttcttgtagaggctgaacgtcttcaaaacaaccttccctgtgctcttgtcgaagatggcttcctcccagtcctccaagttctgcacagccacaaacaggcagcctgtgacgtagaagagcttccagcccaggctatcaaccagcagggaccaggaccggatgcctggagccctcttcagatggaggcgggagctggtgcgggtctccacctgcaggtacatcccgagagggcagcaccactctctacaggaggaggggtctggtctctgtggttgggcacgtcactggatcccccagagaccccgtttcctgtgtaaggaaggcccttttccgttcacagcgacaccgactgcgcgggggctgtttcccgctcagactcacgagctacagctgcatcaccacctgccccgtcctgtctggaaaccttatgtcct

SEQ ID NO: 18934 - RNA, 1651 nt, Homo sapiens
  source 1..1651: mol_type = other RNA
tgcggggacaggccagggcatcaggccaggcgcgctcggtgcacaccgcacctgggaggacctgggtacactcaggagaccaagagcactggcgggtcaggatggttggcgttcagctcctacggggtggggagaagtctgtagccgagagcccagccccctcctgccaggtcttcccaggttcgagagaggctggaactcaatttctgcagaaaatctcccagtttttcctgtttggttagtttttttacaaagacaggatcttgctgtgttgcccaggctggtcttgaactcctggcctcaagcaatcctcccacctcggcctccgaaagtgctgggattactggcatgaaccactgcgcccggctggagctcccggtttttaagcactgcacgatactagaagagctgaccttttttctggcctcacagcttatgctgaagctgagtgtgaggaacagagagacctttctgtgacgaccgctggggcagagtggtctatgcgccgagatcctggcatcagcaagggaggcgggtcctcggggaggggcagcttccacagtgtggctgcagcgtgcacagccaggtaggccctggatgttcacccctcactgcccttggggaagcacctgaccgctggggatgtccaccagggagaggacgctgtgtcggggacaacatgcagcatcagcacccacaagggcccggcctggccccgcctctccactcgcccgaggtcttgctgtggcccaaagcaggagtccagggctggcgagacctccggctgcagaaaggcaggcccaggcctcacgatggagaaagtctggatgtcctggtctggcctgctgtttcatgcagtgtgcaagcagcagcatgagcaggcaataggccaactcggctggaggcaccaactgaagccaaggccacgggtcctgtgggcggtgcacgggctcaggcacaccgggaatgtgccacgggtcctgtgggcggtgcacgggctcaggcacaccgggaatgtgccacgggtcctgtgggcggtgcacgggctcaggcacaccgggaatgtgccacgggtcctgtgggcggtgcacgggctcaggcacaccgggaatgtgccatgggtcctgtgggcggtgcacgggctcaggcacagtggggctgtcagctctggcttgcagggtcaccggcctcactgtcgctgctctgagacagctctgtggggctctcaaggcagtgcagctccaggaagctggtgatgagcttggcgatggcttccacatcactgcggtggcccatgactgcactctgcgtgagggggtgggagaagcccgtcgcaagccggagcaccaccatgtagcctttcccgaagtaccggaccttctcctcctccacgctcacatcacggacatcatggagcaggaccaccacctggtcgtggccagctctgaaaagagtcagcagcttcttgtagaggctgaacgtcttcaaaacaaccttccctgtgctcttgtcgaagatggcttcctcccagtcctccaagttctgcacagccacaaacaggcagcctgtgacgtagaagagcttccagcccaggctatcgagagcacagcggtccccgcgccgcagcagagagacgcgaaccggcgggggc

SEQ ID NO: 18935 - RNA, 1816 nt, Homo sapiens
  source 1..1816: mol_type = other RNA
tgcggggacaggccagggcatcaggccaggcgcgctcggtgcacaccgcacctgggaggacctgggtacactcaggagaccaagagcactggcgggtcaggatggttggcgttcagctcctacggggtggggagaagtctgtagccgagagcccagccccctcctgccaggtcttcccaggttcgagagaggctggaactcaatttctgcagaaaatctcccagtttttcctgtttggttagtttttttacaaagacaggatcttgctgtgttgcccaggctggtcttgaactcctggcctcaagcaatcctcccacctcggcctccgaaagtgctgggattactggcatgaaccactgcgcccggctggagctcccggtttttaagcactgcacgatactagaagagctgaccttttttctggcctcacagcttatgctgaagctgagtgtgaggaacagagagacctttctgtgacgaccgctggggcagagtggtctatgcgccgagatcctggcatcagcaagggaggcgggtcctcggggaggggcagcttccacagtgtggctgcagcgtgcacagccaggtaggccctggatgttcacccctcactgcccttggggaagcacctgaccgctggggatgtccaccagggagaggacgctgtgtcggggacaacatgcagcatcagcacccacaagggcccggcctggccccgcctctccactcgcccgaggtcttgctgtggcccaaagcaggagtccagggctggcgagacctccggctgcagaaaggcaggcccaggcctcacgatggagaaagtctggatgtcctggtctggcctgctgtttcatgcagtgtgcaagcagcagcatgagcaggcaataggccaactcggctggaggcaccaactgaagccaaggccacgggtcctgtgggcggtgcacgggctcaggcacaccgggaatgtgccacgggtcctgtgggcggtgcacgggctcaggcacaccgggaatgtgccacgggtcctgtgggcggtgcacgggctcaggcacaccgggaatgtgccacgggtcctgtgggcggtgcacgggctcaggcacaccgggaatgtgccatgggtcctgtgggcggtgcacgggctcaggcacagtggggctgtcagctctggcttgcagggtcaccggcctcactgtcgctgctctgagacagctctgtggggctctcaaggcagtgcagctccaggaagctggtgatgagcttggcgatggcttccacatcactgcggtggcccatgactgcactctgcgtgagggggtgggagaagcccgtcgcaagccggagcaccaccatgtagcctttcccgaagtaccggaccttctcctcctccacgctcacatcacggacatcatggagcaggaccaccacctggtcgtggccagctctgaaaagagtcagcagcttcttgtagaggctgaacgtcttcaaaacaaccttccctgtgctcttgtcgaagatggcttcctcccagtcctccaagttctgcacagccacaaacaggcagcctgtgacgtagaagagcttccagcccaggctatctccgctgtagtaggcagcagccaggccaatcgacaagattccaaccagcagggaccaggaccggatgcctggagccctcttcagatggaggcgggagctggtgcgggtctccacctgcaggtacatcccgagagggcagcaccactctctacaggaggaggggtcgagagcacagcggtccccgcgccgcagcagagagacgcgaaccggcgggggc

SEQ ID NO: 18936 - RNA, 2036 nt, Homo sapiens
  source 1..2036: mol_type = other RNA
tgcggggacaggccagggcatcaggccaggcgcgctcggtgcacaccgcacctgggaggacctgggtacactcaggagaccaagagcactggcgggtcaggatggttggcgttcagctcctacggggtggggagaagtctgtagccgagagcccagccccctcctgccaggtcttcccaggttcgagagaggctggaactcaatttctgcagaaaatctcccagtttttcctgtttggttagtttttttacaaagacaggatcttgctgtgttgcccaggctggtcttgaactcctggcctcaagcaatcctcccacctcggcctccgaaagtgctgggattactggcatgaaccactgcgcccggctggagctcccggtttttaagcactgcacgatactagaagagctgaccttttttctggcctcacagcttatgctgaagctgagtgtgaggaacagagagacctttctgtgacgaccgctggggcagagtggtctatgcgccgagatcctggcatcagcaagggaggcgggtcctcggggaggggcagcttccacagtgtggctgcagcgtgcacagccaggtaggccctggatgttcacccctcactgcccttggggaagcacctgaccgctggggatgtccaccagggagaggacgctgtgtcggggacaacatgcagcatcagcacccacaagggcccggcctggccccgcctctccactcgcccgaggtcttgctgtggcccaaagcaggagtccagggctggcgagacctccggctgcagaaaggcaggcccaggcctcacgatggagaaagtctggatgtcctggtctggcctgctgtttcatgcagtgtgcaagcagcagcatgagcaggcaataggccaactcggctggaggcaccaactgaagccaaggccacgggtcctgtgggcggtgcacgggctcaggcacaccgggaatgtgccacgggtcctgtgggcggtgcacgggctcaggcacaccgggaatgtgccacgggtcctgtgggcggtgcacgggctcaggcacaccgggaatgtgccacgggtcctgtgggcggtgcacgggctcaggcacaccgggaatgtgccatgggtcctgtgggcggtgcacgggctcaggcacagtggggctgtcagctctggcttgcagggtcaccggcctcactgtcgctgctctgagacagctctgtggggctctcaaggcagtgcagctccaggaagctggtgatgagcttggcgatggcttccacatcactgcggtggcccatgactgcactctgcgtgagggggtgggagaagcccgtcgcaagccggagcaccaccatgtagcctttcccgaagtaccggaccttctcctcctccacgctcacatcacggacatcatggagcaggaccaccacctggtcgtggccagctctgaaaagagtcagcagcttcttgtagaggctgaacgtcttcaaaacaaccttccctgtgctcttgtcgaagatggcttcctcccagtcctccaagttctgcacagccacaaacaggcagcctgtgacgtagaagagcttccagcccaggctatctccgctgtagtaggcagcagccaggccaatcgacaagattccaaccagcagggaccaggaccggatgcctggagccctcttcagatggaggcgggagctggtgcgggtctccacctgcaggtacatcccgagagggcagcaccactctctacaggaggaggggtcgagcgctcgtttctttgtccggatcgggggcgctcccgccgccggggccaacctgcagcggaacaggcgcgaggccgcccgcgacgggcacggcgggacacggaacagccggcaggcgggcccaggacgcagacccctcccggagtgggcctaagggtgccgggacgcgcggcacggagcgggaaggaagtgcggagcccacccagcccagccgcctaccgagagcacagcggtccccgcgccgcagcagagagacgcgaaccggcgggggc

SEQ ID NO: 18937 - RNA, 1866 nt, Homo sapiens
  source 1..1866: mol_type = other RNA
tgcggggacaggccagggcatcaggccaggcgcgctcggtgcacaccgcacctgggaggacctgggtacactcaggagaccaagagcactggcgggtcaggatggttggcgttcagctcctacggggtggggagaagtctgtagccgagagcccagccccctcctgccaggtcttcccaggttcgagagaggctggaactcaatttctgcagaaaatctcccagtttttcctgtttggttagtttttttacaaagacaggatcttgctgtgttgcccaggctggtcttgaactcctggcctcaagcaatcctcccacctcggcctccgaaagtgctgggattactggcatgaaccactgcgcccggctggagctcccggtttttaagcactgcacgatactagaagagctgaccttttttctggcctcacagcttatgctgaagctgagtgtgaggaacagagagacctttctgtgacgaccgctggggcagagtggtctatgcgccgagatcctggcatcagcaagggaggcgggtcctcggggaggggcagcttccacagtgtggctgcagcgtgcacagccaggtaggccctggatgttcacccctcactgcccttggggaagcacctgaccgctggggatgtccaccagggagaggacgctgtgtcggggacaacatgcagcatcagcacccacaagggcccggcctggccccgcctctccactcgcccgaggtcttgctgtggcccaaagcaggagtccagggctggcgagacctccggctgcagaaaggcaggcccaggcctcacgatggagaaagtctggatgtcctggtctggcctgctgtttcatgcagtgtgcaagcagcagcatgagcaggcaataggccaactcggctggaggcaccaactgaagccaaggccacgggtcctgtgggcggtgcacgggctcaggcacaccgggaatgtgccacgggtcctgtgggcggtgcacgggctcaggcacaccgggaatgtgccacgggtcctgtgggcggtgcacgggctcaggcacaccgggaatgtgccacgggtcctgtgggcggtgcacgggctcaggcacaccgggaatgtgccatgggtcctgtgggcggtgcacgggctcaggcacagtggggctgtcagctctggcttgcagggtcaccggcctcactgtcgctgctctgagacagctctgtggggctctcaaggcagtgcagctccaggaagctggtgatgagcttggcgatggcttccacatcactgcggtggcccatgactgcactctgcgtgagggggtgggagaagcccgtcgcaagccggagcaccaccatgtagcctttcccgaagtaccggaccttctcctcctccacgctcacatcacggacatcatggagcaggaccaccacctggtcgtggccagctctgaaaagagtcagcagcttcttgtagaggctgaacgtcttcaaaacaaccttccctgtgctcttgtcgaagatggcttcctcccagtcctccaagttctgcacagccacaaacaggcagcctgtgacgtagaagagcttccagcccaggctatctccgctgtagtaggcagcagccaggccaatcgacaagattccaaccagcagggaccaggaccggatgcctggagccctcttcagatggaggcgggagctggtgcgggtctccacctgcaggtacatcccgagagggcagcaccactctctacaggaggaggggtctggtctctgtggttgggcacgtcactggatcccccagagaccccgtttccgagagcacagcggtccccgcgccgcagcagagagacgcgaaccggcgggggc

SEQ ID NO: 18938 - RNA, 2086 nt, Homo sapiens
  source 1..2086: mol_type = other RNA
tgcggggacaggccagggcatcaggccaggcgcgctcggtgcacaccgcacctgggaggacctgggtacactcaggagaccaagagcactggcgggtcaggatggttggcgttcagctcctacggggtggggagaagtctgtagccgagagcccagccccctcctgccaggtcttcccaggttcgagagaggctggaactcaatttctgcagaaaatctcccagtttttcctgtttggttagtttttttacaaagacaggatcttgctgtgttgcccaggctggtcttgaactcctggcctcaagcaatcctcccacctcggcctccgaaagtgctgggattactggcatgaaccactgcgcccggctggagctcccggtttttaagcactgcacgatactagaagagctgaccttttttctggcctcacagcttatgctgaagctgagtgtgaggaacagagagacctttctgtgacgaccgctggggcagagtggtctatgcgccgagatcctggcatcagcaagggaggcgggtcctcggggaggggcagcttccacagtgtggctgcagcgtgcacagccaggtaggccctggatgttcacccctcactgcccttggggaagcacctgaccgctggggatgtccaccagggagaggacgctgtgtcggggacaacatgcagcatcagcacccacaagggcccggcctggccccgcctctccactcgcccgaggtcttgctgtggcccaaagcaggagtccagggctggcgagacctccggctgcagaaaggcaggcccaggcctcacgatggagaaagtctggatgtcctggtctggcctgctgtttcatgcagtgtgcaagcagcagcatgagcaggcaataggccaactcggctggaggcaccaactgaagccaaggccacgggtcctgtgggcggtgcacgggctcaggcacaccgggaatgtgccacgggtcctgtgggcggtgcacgggctcaggcacaccgggaatgtgccacgggtcctgtgggcggtgcacgggctcaggcacaccgggaatgtgccacgggtcctgtgggcggtgcacgggctcaggcacaccgggaatgtgccatgggtcctgtgggcggtgcacgggctcaggcacagtggggctgtcagctctggcttgcagggtcaccggcctcactgtcgctgctctgagacagctctgtggggctctcaaggcagtgcagctccaggaagctggtgatgagcttggcgatggcttccacatcactgcggtggcccatgactgcactctgcgtgagggggtgggagaagcccgtcgcaagccggagcaccaccatgtagcctttcccgaagtaccggaccttctcctcctccacgctcacatcacggacatcatggagcaggaccaccacctggtcgtggccagctctgaaaagagtcagcagcttcttgtagaggctgaacgtcttcaaaacaaccttccctgtgctcttgtcgaagatggcttcctcccagtcctccaagttctgcacagccacaaacaggcagcctgtgacgtagaagagcttccagcccaggctatctccgctgtagtaggcagcagccaggccaatcgacaagattccaaccagcagggaccaggaccggatgcctggagccctcttcagatggaggcgggagctggtgcgggtctccacctgcaggtacatcccgagagggcagcaccactctctacaggaggaggggtctggtctctgtggttgggcacgtcactggatcccccagagaccccgtttccgagcgctcgtttctttgtccggatcgggggcgctcccgccgccggggccaacctgcagcggaacaggcgcgaggccgcccgcgacgggcacggcgggacacggaacagccggcaggcgggcccaggacgcagacccctcccggagtgggcctaagggtgccgggacgcgcggcacggagcgggaaggaagtgcggagcccacccagcccagccgcctaccgagagcacagcggtccccgcgccgcagcagagagacgcgaaccggcgggggc

SEQ ID NO: 18939 - RNA, 2033 nt, Homo sapiens
  source 1..2033: mol_type = other RNA
tgcggggacaggccagggcatcaggccaggcgcgctcggtgcacaccgcacctgggaggacctgggtacactcaggagaccaagagcactggcgggtcaggatggttggcgttcagctcctacggggtggggagaagtctgtagccgagagcccagccccctcctgccaggtcttcccaggttcgagagaggctggaactcaatttctgcagaaaatctcccagtttttcctgtttggttagtttttttacaaagacaggatcttgctgtgttgcccaggctggtcttgaactcctggcctcaagcaatcctcccacctcggcctccgaaagtgctgggattactggcatgaaccactgcgcccggctggagctcccggtttttaagcactgcacgatactagaagagctgaccttttttctggcctcacagcttatgctgaagctgagtgtgaggaacagagagacctttctgtgacgaccgctggggcagagtggtctatgcgccgagatcctggcatcagcaagggaggcgggtcctcggggaggggcagcttccacagtgtggctgcagcgtgcacagccaggtaggccctggatgttcacccctcactgcccttggggaagcacctgaccgctggggatgtccaccagggagaggacgctgtgtcggggacaacatgcagcatcagcacccacaagggcccggcctggccccgcctctccactcgcccgaggtcttgctgtggcccaaagcaggagtccagggctggcgagacctccggctgcagaaaggcaggcccaggcctcacgatggagaaagtctggatgtcctggtctggcctgctgtttcatgcagtgtgcaagcagcagcatgagcaggcaataggccaactcggctggaggcaccaactgaagccaaggccacgggtcctgtgggcggtgcacgggctcaggcacaccgggaatgtgccacgggtcctgtgggcggtgcacgggctcaggcacaccgggaatgtgccacgggtcctgtgggcggtgcacgggctcaggcacaccgggaatgtgccacgggtcctgtgggcggtgcacgggctcaggcacaccgggaatgtgccatgggtcctgtgggcggtgcacgggctcaggcacagtggggctgtcagctctggcttgcagggtcaccggcctcactgtcgctgctctgagacagctctgtggggctctcaaggcagtgcagctccaggaagctggtgatgagcttggcgatggcttccacatcactgcggtggcccatgactgcactctgcgtgagggggtgggagaagcccgtcgcaagccggagcaccaccatgtagcctttcccgaagtaccggaccttctcctcctccacgctcacatcacggacatcatggagcaggaccaccacctggtcgtggccagctctgaaaagagtcagcagcttcttgtagaggctgaacgtcttcaaaacaaccttccctgtgctcttgtcgaagatggcttcctcccagtcctccaagttctgcacagccacaaacaggcagcctgtgacgtagaagagcttccagcccaggctatctccgctgtagtaggcagcagccaggccaatcgacaagattccaaccagcagggaccaggaccggatgcctggagccctcttcagatggaggcgggagctggtgcgggtctccacctgcaggtacatcccgagagggcagcaccactctctacaggaggaggggtctggtctctgtggttgggcacgtcactggatcccccagagaccccgtttcctgcagcggaacaggcgcgaggccgcccgcgacgggcacggcgggacacggaacagccggcaggcgggcccaggacgcagacccctcccggagtgggcctaagggtgccgggacgcgcggcacggagcgggaaggaagtgcggagcccacccagcccagccgcctaccgagagcacagcggtccccgcgccgcagcagagagacgcgaaccggcgggggc

SEQ ID NO: 18940 - RNA, 2059 nt, Homo sapiens
  source 1..2059: mol_type = other RNA
tgcggggacaggccagggcatcaggccaggcgcgctcggtgcacaccgcacctgggaggacctgggtacactcaggagaccaagagcactggcgggtcaggatggttggcgttcagctcctacggggtggggagaagtctgtagccgagagcccagccccctcctgccaggtcttcccaggttcgagagaggctggaactcaatttctgcagaaaatctcccagtttttcctgtttggttagtttttttacaaagacaggatcttgctgtgttgcccaggctggtcttgaactcctggcctcaagcaatcctcccacctcggcctccgaaagtgctgggattactggcatgaaccactgcgcccggctggagctcccggtttttaagcactgcacgatactagaagagctgaccttttttctggcctcacagcttatgctgaagctgagtgtgaggaacagagagacctttctgtgacgaccgctggggcagagtggtctatgcgccgagatcctggcatcagcaagggaggcgggtcctcggggaggggcagcttccacagtgtggctgcagcgtgcacagccaggtaggccctggatgttcacccctcactgcccttggggaagcacctgaccgctggggatgtccaccagggagaggacgctgtgtcggggacaacatgcagcatcagcacccacaagggcccggcctggccccgcctctccactcgcccgaggtcttgctgtggcccaaagcaggagtccagggctggcgagacctccggctgcagaaaggcaggcccaggcctcacgatggagaaagtctggatgtcctggtctggcctgctgtttcatgcagtgtgcaagcagcagcatgagcaggcaataggccaactcggctggaggcaccaactgaagccaaggccacgggtcctgtgggcggtgcacgggctcaggcacaccgggaatgtgccacgggtcctgtgggcggtgcacgggctcaggcacaccgggaatgtgccacgggtcctgtgggcggtgcacgggctcaggcacaccgggaatgtgccacgggtcctgtgggcggtgcacgggctcaggcacaccgggaatgtgccatgggtcctgtgggcggtgcacgggctcaggcacagtggggctgtcagctctggcttgcagggtcaccggcctcactgtcgctgctctgagacagctctgtggggctctcaaggcagtgcagctccaggaagctggtgatgagcttggcgatggcttccacatcactgcggtggcccatgactgcactctgcgtgagggggtgggagaagcccgtcgcaagccggagcaccaccatgtagcctttcccgaagtaccggaccttctcctcctccacgctcacatcacggacatcatggagcaggaccaccacctggtcgtggccagctctgaaaagagtcagcagcttcttgtagaggctgaacgtcttcaaaacaaccttccctgtgctcttgtcgaagatggcttcctcccagtcctccaagttctgcacagccacaaacaggcagcctgtgacgtagaagagcttccagcccaggctatctccgctgtagtaggcagcagccaggccaatcgacaagattccaaccagcagggaccaggaccggatgcctggagccctcttcagatggaggcgggagctggtgcgggtctccacctgcaggtacatcccgagagggcagcaccactctctacaggaggaggggtctggtctctgtggttgggcacgtcactggatcccccagagaccccgtttcctgtgtaaggaaggcccttttccgttcacagcgacaccgactgcgcgggggctgtttcccgctcagactcacgagctacagctgcatcaccacctgccccgtcctgtctggaaaccttatgtcctgaggccgctagcccccagcagcctttaagcttctagcatctgtgggcaccccctctcccctgtgctggcctccaccaagaaaggaactgaaagtcccatcatggcttccggccgtactggc

SEQ ID NO: 18941 - RNA, 1693 nt, Homo sapiens
  source 1..1693: mol_type = other RNA
tgcggggacaggccagggcatcaggccaggcgcgctcggtgcacaccgcacctgggaggacctgggtacactcaggagaccaagagcactggcgggtcaggatggttggcgttcagctcctacggggtggggagaagtctgtagccgagagcccagccccctcctgccaggtcttcccaggttcgagagaggctggaactcaatttctgcagaaaatctcccagtttttcctgtttggttagtttttttacaaagacaggatcttgctgtgttgcccaggctggtcttgaactcctggcctcaagcaatcctcccacctcggcctccgaaagtgctgggattactggcatgaaccactgcgcccggctggagctcccggtttttaagcactgcacgatactagaagagctgaccttttttctggcctcacagcttatgctgaagctgagtgtgaggaacagagagacctttctgtgacgaccgctggggcagagtggtctatgcgccgagatcctggcatcagcaagggaggcgggtcctcggggaggggcagcttccacagtgtggctgcagcgtgcacagccaggtaggccctggatgttcacccctcactgcccttggggaagcacctgaccgctggggatgtccaccagggagaggacgctgtgtcggggacaacatgcagcatcagcacccacaagggcccggcctggccccgcctctccactcgcccgaggtcttgctgtggcccaaagcaggagtccagggctggcgagacctccggctgcagaaaggcaggcccaggcctcacgatggagaaagtctggatgtcctggtctggcctgctgtttcatgcagtgtgcaagcagcagcatgagcaggcaataggccaactcggctggaggcaccaactgaagccaaggccacgggtcctgtgggcggtgcacgggctcaggcacaccgggaatgtgccacgggtcctgtgggcggtgcacgggctcaggcacaccgggaatgtgccacgggtcctgtgggcggtgcacgggctcaggcacaccgggaatgtgccacgggtcctgtgggcggtgcacgggctcaggcacaccgggaatgtgccatgggtcctgtgggcggtgcacgggctcaggcacagtggggctgtcagctctggcttgcagggtcaccggcctcactgtcgctgctctgagacagctctgtggggctctcaaggcagtgcagctccaggaagctggtgatgagcttggcgatggcttccacatcactgcggtggcccatgactgcactctgcgtgagggggtgggagaagcccgtcgcaagccggagcaccaccatgtagcctttcccgaagtaccggaccttctcctcctccacgctcacatcacggacatcatggagcaggaccaccacctggtcgtggccagctctgaaaagagtcagcagcttcttgtagaggctgaacgtcttcaaaacaaccttccctgtgctcttgtcgaagatggcttcctcccagtcctccaagttctgcacagccacaaacaggcagcctgtgacgtagaagagcttccagcccaggctatctccgctgtagtaggcagcagccaggccaatcgacaagattccgagagcacagcggtccccgcgccgcagcagagagacgcgaaccggcgggggc

SEQ ID NO: 18942 - RNA, 1742 nt, Homo sapiens
  source 1..1742: mol_type = other RNA
tgcggggacaggccagggcatcaggccaggcgcgctcggtgcacaccgcacctgggaggacctgggtacactcaggagaccaagagcactggcgggtcaggatggttggcgttcagctcctacggggtggggagaagtctgtagccgagagcccagccccctcctgccaggtcttcccaggttcgagagaggctggaactcaatttctgcagaaaatctcccagtttttcctgtttggttagtttttttacaaagacaggatcttgctgtgttgcccaggctggtcttgaactcctggcctcaagcaatcctcccacctcggcctccgaaagtgctgggattactggcatgaaccactgcgcccggctggagctcccggtttttaagcactgcacgatactagaagagctgaccttttttctggcctcacagcttatgctgaagctgagtgtgaggaacagagagacctttctgtgacgaccgctggggcagagtggtctatgcgccgagatcctggcatcagcaagggaggcgggtcctcggggaggggcagcttccacagtgtggctgcagcgtgcacagccaggtaggccctggatgttcacccctcactgcccttggggaagcacctgaccgctggggatgtccaccagggagaggacgctgtgtcggggacaacatgcagcatcagcacccacaagggcccggcctggccccgcctctccactcgcccgaggtcttgctgtggcccaaagcaggagtccagggctggcgagacctccggctgcagaaaggcaggcccaggcctcacgatggagaaagtctggatgtcctggtctggcctgctgtttcatgcagtgtgcaagcagcagcatgagcaggcaataggccaactcggctggaggcaccaactgaagccaaggccacgggtcctgtgggcggtgcacgggctcaggcacaccgggaatgtgccacgggtcctgtgggcggtgcacgggctcaggcacaccgggaatgtgccacgggtcctgtgggcggtgcacgggctcaggcacaccgggaatgtgccacgggtcctgtgggcggtgcacgggctcaggcacaccgggaatgtgccatgggtcctgtgggcggtgcacgggctcaggcacagtggggctgtcagctctggcttgcagggtcaccggcctcactgtcgctgctctgagacagctctgtggggctctcaaggcagtgcagctccaggaagctggtgatgagcttggcgatggcttccacatcactgcggtggcccatgactgcactctgcgtgagggggtgggagaagcccgtcgcaagccggagcaccaccatgtagcctttcccgaagtaccggaccttctcctcctccacgctcacatcacggacatcatggagcaggaccaccacctggtcgtggccagctctgaaaagagtcagcagcttcttgtagaggctgaacgtcttcaaaacaaccttccctgtgctcttgtcgaagatggcttcctccgctgtagtaggcagcagccaggccaatcgacaagattccaaccagcagggaccaggaccggatgcctggagccctcttcagatggaggcgggagctggtgcgggtctccacctgcaggtacatcccgagagggcagcaccactctctacaggaggaggggtcgagagcacagcggtccccgcgccgcagcagagagacgcgaaccggcgggggc

SEQ ID NO: 18943 - RNA, 1795 nt, Homo sapiens
  source 1..1795: mol_type = other RNA
tgcggggacaggccagggcatcaggccaggcgcgctcggtgcacaccgcacctgggaggacctgggtacactcaggagaccaagagcactggcgggtcaggatggttggcgttcagctcctacggggtggggagaagtctgtagccgagagcccagccccctcctgccaggtcttcccaggttcgagagaggctggaactcaatttctgcagaaaatctcccagtttttcctgtttggttagtttttttacaaagacaggatcttgctgtgttgcccaggctggtcttgaactcctggcctcaagcaatcctcccacctcggcctccgaaagtgctgggattactggcatgaaccactgcgcccggctggagctcccggtttttaagcactgcacgatactagaagagctgaccttttttctggcctcacagcttatgctgaagctgagtgtgaggaacagagagacctttctgtgacgaccgctggggcagagtggtctatgcgccgagatcctggcatcagcaagggaggcgggtcctcggggaggggcagcttccacagtgtggctgcagcgtgcacagccaggtaggccctggatgttcacccctcactgcccttggggaagcacctgaccgctggggatgtccaccagggagaggacgctgtgtcggggacaacatgcagcatcagcacccacaagggcccggcctggccccgcctctccactcgcccgaggtcttgctgtggcccaaagcaggagtccagggctggcgagacctccggctgcagaaaggcaggcccaggcctcacgatggagaaagtctggatgtcctggtctggcctgctgtttcatgcagtgtgcaagcagcagcatgagcaggcaataggccaactcggctggaggcaccaactgaagccaaggccacgggtcctgtgggcggtgcacgggctcaggcacaccgggaatgtgccacgggtcctgtgggcggtgcacgggctcaggcacaccgggaatgtgccacgggtcctgtgggcggtgcacgggctcaggcacaccgggaatgtgccatgggtcctgtgggcggtgcacgggctcaggcacagtggggctgtcagctctggcttgcagggtcaccggcctcactgtcgctgctctgagacagctctgtggggctctcaaggcagtgcagctccaggaagctggtgatgagcttggcgatggcttccacatcactgcggtggcccatgactgcactctgcgtgagggggtgggagaagcccgtcgcaagccggagcaccaccatgtagcctttcccgaagtaccggaccttctcctcctccacgctcacatcacggacatcatggagcaggaccaccacctggtcgtggccagctctgaaaagagtcagcagcttcttgtagaggctgaacgtcttcaaaacaaccttccctgtgctcttgtcgaagatggcttcctcccagtcctccaagttctgcacagccacaaacaggcagcctgtgacgtagaagagcttccagcccaggctatcaaccagcagggaccaggaccggatgcctggagccctcttcagatggaggcgggagctggtgcgggtctccacctgcaggtacatcccgagagggcagcaccactctctacaggaggaggggtcgagagcacagcggtccccgcgccgcagcagagagacgcgaaccggcgggggcggggccgcgcgcacttccgggattggagcggagccgagccgactttcgggggcggggccgcgcgcgctt

SEQ ID NO: 18944 - RNA, 1792 nt, Homo sapiens
  source 1..1792: mol_type = other RNA
tgcggggacaggccagggcatcaggccaggcgcgctcggtgcacaccgcacctgggaggacctgggtacactcaggagaccaagagcactggcgggtcaggatggttggcgttcagctcctacggggtggggagaagtctgtagccgagagcccagccccctcctgccaggtcttcccaggttcgagagaggctggaactcaatttctgcagaaaatctcccagtttttcctgtttggttagtttttttacaaagacaggatcttgctgtgttgcccaggctggtcttgaactcctggcctcaagcaatcctcccacctcggcctccgaaagtgctgggattactggcatgaaccactgcgcccggctggagctcccggtttttaagcactgcacgatactagaagagctgaccttttttctggcctcacagcttatgctgaagctgagtgtgaggaacagagagacctttctgtgacgaccgctggggcagagtggtctatgcgccgagatcctggcatcagcaagggaggcgggtcctcggggaggggcagcttccacagtgtggctgcagcgtgcacagccaggtaggccctggatgttcacccctcactgcccttggggaagcacctgaccgctggggatgtccaccagggagaggacgctgtgtcggggacaacatgcagcatcagcacccacaagggcccggcctggccccgcctctccactcgcccgaggtcttgctgtggcccaaagcaggagtccagggctggcgagacctccggctgcagaaaggcaggcccaggcctcacgatggagaaagtctggatgtcctggtctggcctgctgtttcatgcagtgtgcaagcagcagcatgagcaggcaataggccaactcggctggaggcaccaactgaagccaaggccacgggtcctgtgggcggtgcacgggctcaggcacaccgggaatgtgccacgggtcctgtgggcggtgcacgggctcaggcacaccgggaatgtgccacgggtcctgtgggcggtgcacgggctcaggcacaccgggaatgtgccatgggtcctgtgggcggtgcacgggctcaggcacagtggggctgtcagctctggcttgcagggtcaccggcctcactgtcgctgctctgagacagctctgtggggctctcaaggcagtgcagctccaggaagctggtgatgagcttggcgatggcttccacatcactgcggtggcccatgactgcactctgcgtgagggggtgggagaagcccgtcgcaagccggagcaccaccatgtagcctttcccgaagtaccggaccttctcctcctccacgctcacatcacggacatcatggagcaggaccaccacctggtcgtggccagctctgaaaagagtcagcagcttcttgtagaggctgaacgtcttcaaaacaaccttccctgtgctcttgtcgaagatggcttcctcccagtcctccaagttctgcacagccacaaacaggcagcctgtgacgtagaagagcttccagcccaggctatctccgctgtagtaggcagcagccaggccaatcgacaagattccaaccagcagggaccaggaccggatgcctggagccctcttcagatggaggcgggagctggtgcgggtctccacctgcaggtacatcccgagagggcagcaccactctctacaggaggaggggtcgagagcacagcggtccccgcgccgcagcagagagacgcgaaccggcgggggcggggccgcgcgcacttccgggatt

SEQ ID NO: 18945 - RNA, 2006 nt, Homo sapiens
  source 1..2006: mol_type = other RNA
tgcggggacaggccagggcatcaggccaggcgcgctcggtgcacaccgcacctgggaggacctgggtacactcaggagaccaagagcactggcgggtcaggatggttggcgttcagctcctacggggtggggagaagtctgtagccgagagcccagccccctcctgccaggtcttcccaggttcgagagaggctggaactcaatttctgcagaaaatctcccagtttttcctgtttggttagtttttttacaaagacaggatcttgctgtgttgcccaggctggtcttgaactcctggcctcaagcaatcctcccacctcggcctccgaaagtgctgggattactggcatgaaccactgcgcccggctggagctcccggtttttaagcactgcacgatactagaagagctgaccttttttctggcctcacagcttatgctgaagctgagtgtgaggaacagagagacctttctgtgacgaccgctggggcagagtggtctatgcgccgagatcctggcatcagcaagggaggcgggtcctcggggaggggcagcttccacagtgtggctgcagcgtgcacagccaggtaggccctggatgttcacccctcactgcccttggggaagcacctgaccgctggggatgtccaccagggagaggacgctgtgtcggggacaacatgcagcatcagcacccacaagggcccggcctggccccgcctctccactcgcccgaggtcttgctgtggcccaaagcaggagtccagggctggcgagacctccggctgcagaaaggcaggcccaggcctcacgatggagaaagtctggatgtcctggtctggcctgctgtttcatgcagtgtgcaagcagcagcatgagcaggcaataggccaactcggctggaggcaccaactgaagccaaggccacgggtcctgtgggcggtgcacgggctcaggcacaccgggaatgtgccacgggtcctgtgggcggtgcacgggctcaggcacaccgggaatgtgccacgggtcctgtgggcggtgcacgggctcaggcacaccgggaatgtgccatgggtcctgtgggcggtgcacgggctcaggcacagtggggctgtcagctctggcttgcagggtcaccggcctcactgtcgctgctctgagacagctctgtggggctctcaaggcagtgcagctccaggaagctggtgatgagcttggcgatggcttccacatcactgcggtggcccatgactgcactctgcgtgagggggtgggagaagcccgtcgcaagccggagcaccaccatgtagcctttcccgaagtaccggaccttctcctcctccacgctcacatcacggacatcatggagcaggaccaccacctggtcgtggccagctctgaaaagagtcagcagcttcttgtagaggctgaacgtcttcaaaacaaccttccctgtgctcttgtcgaagatggcttcctcccagtcctccaagttctgcacagccacaaacaggcagcctgtgacgtagaagagcttccagcccaggctatctccgctgtagtaggcagcagccaggccaatcgacaagattccaaccagcagggaccaggaccggatgcctggagccctcttcagatggaggcgggagctggtgcgggtctccacctgcaggtacatcccgagagggcagcaccactctctacaggaggaggggtcgagcgctcgtttctttgtccggatcgggggcgctcccgccgccggggccaacctgcagcggaacaggcgcgaggccgcccgcgacgggcacggcgggacacggaacagccggcaggcgggcccaggacgcagacccctcccggagtgggcctaagggtgccgggacgcgcggcacggagcgggaaggaagtgcggagcccacccagcccagccgcctaccgagagcacagcggtccccgcgccgcagcagagagacgcgaaccggcgggggcggggccgcgcgcacttcc

SEQ ID NO: 18946 - RNA, 2896 nt, Homo sapiens
  source 1..2896: mol_type = other RNA
tgcggggacaggccagggcatcaggccaggcgcgctcggtgcacaccgcacctgggaggacctgggtacactcaggagaccaagagcactggcgggtcaggatggttggcgttcagctcctacggggtggggagaagtctgtagccgagagcccagccccctcctgccaggtcttcccaggttcgagagaggctggaactcaatttctgcagaaaatctcccagtttttcctgtttggttagtttttttacaaagacaggatcttgctgtgttgcccaggctggtcttgaactcctggcctcaagcaatcctcccacctcggcctccgaaagtgctgggattactggcatgaaccactgcgcccggctggagctcccggtttttaagcactgcacgatactagaagagctgaccttttttctggcctcacagcttatgctgaagctgagtgtgaggaacagagagacctttctgtgacgaccgctggggcagagtggtctatgcgccgagatcctggcatcagcaagggaggcgggtcctcggggaggggcagcttccacagtgtggctgcagcgtgcacagccaggtaggccctggatgttcacccctcactgcccttggggaagcacctgaccgctggggatgtccaccagggagaggacgctgtgtcggggacaacatgcagcatcagcacccacaagggcccggcctggccccgcctctccactcgcccgaggtcttgctgtggcccaaagcaggagtccagggctggcgagacctccggctgcagaaaggcaggcccaggcctcacgatggagaaagtctggatgtcctggtctggcctgctgtttcatgcagtgtgcaagcagcagcatgagcaggcaataggccaactcggctggaggcaccaactgaagccaaggccacgggtcctgtgggcggtgcacgggctcaggcacaccgggaatgtgccacgggtcctgtgggcggtgcacgggctcaggcacaccgggaatgtgccacgggtcctgtgggcggtgcacgggctcaggcacaccgggaatgtgccatgggtcctgtgggcggtgcacgggctcaggcacagtggggctgtcagctctggcttgcagggtcaccggcctcactgtcgctgctctgagacagctctgtggggctctcaaggcagtgcagctccaggaagctggtgatgagcttggcgatggcttccacatcactgcggtggcccatgactgcactctgcgtgagggggtgggagaagcccgtcgcaagccggagcaccaccatgtagcctttcccgaagtaccggaccttctcctcctccacgctcacatcacggacatcatggagcaggaccaccacctggtcgtggccagctctgaaaagagtcagcagcttcttgtagaggctgaacgtcttcaaaacaaccttccctgtgctcttgtcgaagatggcttcctcccagtcctccaagttctgcacagccacaaacaggcagcctgtgacgtagaagagcttccagcccaggctatctccgctgtagtaggcagcagccaggccaatcgacaagattccaaccagcagggaccaggaccggatgcctggagccctcttcagatggaggcgggagctggtgcgggtctccacctgcaggtacatcccgagagggcagcaccactctctacaggaggaggggtctgggaacagacagaggcagctgagcccttgggcctgcacacaggcaggcgcccacgccatcaggcccagtctggaggccaagagcaggtcccccaactaagtcacctgcagccccagacaccatcagccagtctcacctggtctctgtggttgggcacgtcactggatcccccagagaccccgtttcctgtgtaaggaaggcccttttccgttcacagcgacaccgactgcgcgggggctgtttcccgctcagactcacgagctacagctgcatcaccacctgccccgtcctgtctggaaaccttatgtcctgaggccgctagcccccagcagcctttaagcttctagcatctgtgggcaccccctctcccctgtgctggcctccaccaagaaaggaactgaaagtcccatcatggcttccggccgtactggctctcgcactggcatggaccaacgatctcagctctctctctgccctcctccacctgctgaaagttcagactgcacagtagagggtcccaaagcggccagaaccgacgagtcaccaaaggggctaatcttccacagcggagttccgcacgggcgcagcagccctgccacttcaccgtacgctcccaacactggccccagggaccccgttctggtagtttctcagggctttccctgtgaagtcaaatcaaatttctgacattaagtagggggttcaggctgggcgcggtggctcaggcctgtaatctcagcactttgggaggacgaggcgtgcggattgtttgagtcacggagttcaagaccagccagggcaacgtggcgaaaccccgtctccacagaaaatacataaaacagcccggtgtggtggtgtacgcctgtggtcctagttattcaggaggctgagctgggaggatcacctgaggccgggaggtggaggctgcagtgagcagaaatcgtgccactggactccagcctgggtgacagagtgagaccgtgtctcaaaaaaataaaaaatagtgggttcaaatcacacaaaccaatcctagatgctggtatatgactgggctccctcccgggcctcagttgcctcattgctcccgaaacacccggcattccacatccaaatgcacacacacacgcacactcgcggacacaagcacacgcgcgctggcaaagccgcccgcgccgctag

SEQ ID NO: 18947 - RNA, 1842 nt, Homo sapiens
  source 1..1842: mol_type = other RNA
tgcggggacaggccagggcatcaggccaggcgcgctcggtgcacaccgcacctgggaggacctgggtacactcaggagaccaagagcactggcgggtcaggatggttggcgttcagctcctacggggtggggagaagtctgtagccgagagcccagccccctcctgccaggtcttcccaggttcgagagaggctggaactcaatttctgcagaaaatctcccagtttttcctgtttggttagtttttttacaaagacaggatcttgctgtgttgcccaggctggtcttgaactcctggcctcaagcaatcctcccacctcggcctccgaaagtgctgggattactggcatgaaccactgcgcccggctggagctcccggtttttaagcactgcacgatactagaagagctgaccttttttctggcctcacagcttatgctgaagctgagtgtgaggaacagagagacctttctgtgacgaccgctggggcagagtggtctatgcgccgagatcctggcatcagcaagggaggcgggtcctcggggaggggcagcttccacagtgtggctgcagcgtgcacagccaggtaggccctggatgttcacccctcactgcccttggggaagcacctgaccgctggggatgtccaccagggagaggacgctgtgtcggggacaacatgcagcatcagcacccacaagggcccggcctggccccgcctctccactcgcccgaggtcttgctgtggcccaaagcaggagtccagggctggcgagacctccggctgcagaaaggcaggcccaggcctcacgatggagaaagtctggatgtcctggtctggcctgctgtttcatgcagtgtgcaagcagcagcatgagcaggcaataggccaactcggctggaggcaccaactgaagccaaggccacgggtcctgtgggcggtgcacgggctcaggcacaccgggaatgtgccacgggtcctgtgggcggtgcacgggctcaggcacaccgggaatgtgccacgggtcctgtgggcggtgcacgggctcaggcacaccgggaatgtgccatgggtcctgtgggcggtgcacgggctcaggcacagtggggctgtcagctctggcttgcagggtcaccggcctcactgtcgctgctctgagacagctctgtggggctctcaaggcagtgcagctccaggaagctggtgatgagcttggcgatggcttccacatcactgcggtggcccatgactgcactctgcgtgagggggtgggagaagcccgtcgcaagccggagcaccaccatgtagcctttcccgaagtaccggaccttctcctcctccacgctcacatcacggacatcatggagcaggaccaccacctggtcgtggccagctctgaaaagagtcagcagcttcttgtagaggctgaacgtcttcaaaacaaccttccctgtgctcttgtcgaagatggcttcctcccagtcctccaagttctgcacagccacaaacaggcagcctgtgacgtagaagagcttccagcccaggctatctccgctgtagtaggcagcagccaggccaatcgacaagattccaaccagcagggaccaggaccggatgcctggagccctcttcagatggaggcgggagctggtgcgggtctccacctgcaggtacatcccgagagggcagcaccactctctacaggaggaggggtctggtctctgtggttgggcacgtcactggatcccccagagaccccgtttccgagagcacagcggtccccgcgccgcagcagagagacgcgaaccggcgggggcggggccgcgcgcacttccgggatt

SEQ ID NO: 18948 - RNA, 2296 nt, Homo sapiens
  source 1..2296: mol_type = other RNA
tgcggggacaggccagggcatccctgaatgtcaagtatttgtttcacccgctgtcctgtaggactgtcggcaatagtgaagccgaagccctgggcacctttcacaatggttaaggtcataagttcagcttgggtggccccagatgaagccatagacacattgtcatcatggacgggcggtggatacgtgccgtctagctgaccatcagttggcatggagtgcagagaatgaggcggccgatctgttatatctggaactgactgtgaggtccgagaaatgtactccaaatatgtttcatagttgtgtcttccattgaccatcactggaggtggcctctccattattgcaaggggtggcaccatgctgttagcagggtcttcaggatcaaagggcaaagggtagccacgacacaacaccaggttgacactctgaccaataggaacagactggaaaagtttgacaacatctgcatgagtgtgtccaaggacacaaacttcattaatatagacaatgacatcacctgtttccatttttccatcctgtgctgcaggcccatccggaatcacacttttcacctgcagaaactcatcaggctcgtctccaccaatgatggtaaatccaaagcccatgttgctcttttttagggtggtgctgaggaatgttcccttcaactgggatgcatcccgggtgaagagtggtttttcgaacagccagggcctccctgctgggtcgcgctgatagtaagacaagtcattcacgctgcgcgacctctccggggcagcacgggggcggatggatttgggcctaggtaatgtccatgaggagctgtctactcggaaacctggggcctgcaggggctttgttccaagttctgtgtggggcatgttatgttgctgtagcttcctttttgcttccaggacaggattttcaaactgtgttcttctatttatgtggtcaacataataagtgccataaatgggatcatcgattttttcccagccatatggaagctcattttctttgcactcttctggaggtttagcctttttcgcaagtcgtggatccagccatgatgttgtctttgtgttatggtcaatgaagtagacttcgcccttctctgtataggccatttcccagttatcaggcaatgggtctggttcctcattgtcttcaggtttagttggctttgtgtcatccatctgctccttcagctcctcaggctgactgtacactggtgcaggataaggctgggagggcatctcccctgaggcacctgcacttttgtcttcatgttcactggattctggtgttactactactccatttccattgaccacaggcctctcttcctcttcctcctcaggaggctctatactggctttctccatgttgctcactgatttattcctcttccgttttccttcagcacttggagtggctcctggaagtatctggtctgttacatttaacaataatggtgctggttctgctggcggctttggggtaccgtagtaattgtcttcataagtcccactttctaggagagcaccacttttctccaattccataaaatcttcaacagtgatgaaaatataatccactccagggacctcaccctccttatgtggccttgtggtgcatggcaccgtgcggaggtagaggttgtcacgaatgatttgctgaagctcatggtccacagaacccttttgaaatcgtaagttgaggtagtgacgaaggtctttatcaacaattcctccttgcttgacacacttgagccggagggggtccttgcagtgtttgatcacggccagcacgtccctgatggtgagccccgccacgggggtctcgttcacctccagcagcagctcctccgacaccaatttgctgccgctctcataggccaccttgccgggcttcacctcccccaggtaggggaactgtccattctcggcgccccccttcagttcaaagcccagctggccctccgggttcctgccaatgacactctcatggactttgctagtccagtggcttttctttttcaagcttttggacatggcagtggggcgagtcgcctcagttcctgggctccttggggttaggggggctggtggtgagagaatgaggatggaggagcaagggggcccagggggaagaacagcagactttgccttcgcccccctctattcggtgctttccctcttctttggatggagtgtggacgaggaatggggaggatgagagggacggctgggcagaggtaggagagcttggatgaggttgtgctgtcccttga

SEQ ID NO: 18949 - RNA, 5859 nt, Homo sapiens
  source 1..5859: mol_type = other RNA
tgcggggacaggccagggcatccctgaatgtcaagtatttgtttcacccgctgtcctgtaggactgtcggcaatagtgaagccgaagccctgggcacctttcacaatggttaaggtcataagttcagcttgggtggccccagatgaagccatagacacattgtcatcatggacgggcggtggatacgtgccgtctagctgaccatcagttggcatggagtgcagagaatgaggcggccgatctgttatatctggaactgactgtgaggtccgagaaatgtactccaaatatgtttcatagttgtgtcttccattgaccatcactggaggtggcctctccattattgcaaggggtggcaccatgctgttagcagggtcttcaggatcaaagggcaaagggtagccacgacacaacaccaggttgacactctgaccaataggaacagactggaaaagtttgacaacatctgcatgagtgtgtccaaggacacaaacttcattaatatagacaatgacatcacctgtttccatttttccatcctgtgctgcaggcccatccggaatcacacttttcacctgcagaaactcatcaggctcgtctccaccaatgatggtaaatccaaagcccatgttgctcttttttagggtggtgctgaggaatgttcccttcaactgggatgcatcccgggtgaagagtggtttttcgaacagccagggcctccctgctgggtcgcgctgatagtaagacaagtcattcacgctgcgcgacctctccggggcagcacgggggcggatggatttgggcctaggtaatgtccatgaggagctgtctactcggaaacctggggcctgcaggggctttgttccaagttctgtgtggggcatgttatgttgctgtagcttcctttttgcttccaggacaggattttcaaactgtgttcttctatttatgtggtcaacataataagtgccataaatgggatcatcgattttttcccagccatatggaagctcattttctttgcactcttctggaggtttagcctttttcgcaagtcgtggatccagccatgatgttgtctttgtgttatggtcaatgaagtagacttcgcccttctctgtataggccatttcccagttatcaggcaatgggtctggttcctcattgtcttcaggtttagttggctttgtgtcatccatctgctccttcagctcctcaggctgactgtacactggtgcaggataaggctgggagggcatctcccctgaggcacctgcacttttgtcttcatgttcactggattctggtgttactactactccatttccattgaccacaggcctctcttcctcttcctcctcaggaggctctatactggctttctccatgttgctcactgatttattcctcttccgttttccttcagcacttggagtggctcctggaagtatctggtctgttacatttaacaataatggtgctggttctgctggcggctttggggtaccgtagtaattgtcttcataagtcccactttctaggagagcaccacttttctccaattccataaaatcttcaacagtgatgaaaatataatccactccagggacctcaccctccttatgtggccttgtggtgcctagagctctgttcaaaggaagcagagaagccgcacgtcctctcccacctttccatggtcctcagtcagtgtcttctcaaaccacctgtactgatccaacccattcgcagataaaaataattttcttgatagaagtagtctcagctgagctttgatttttcaacatggatgtctagaattttcctctttaagccagacacagcaacacaaaactgccgctgagctcttttgttttccctcctctcaaagatgaagcatgcagcacttctctctctctctctctgtctccctctgcctctccctctctccctctccctctctctccttctcccctctctcgcttatgctctctccctccgtttccctttccccaacccccaccagcaacctcgctcgcttcccggtcagtcaggggcatttacatctctcagcacaagaacctgtgttatctacgcgcctgtctctcacttttgggtttcctctgggaaagggaggggggcggctctaggtgaagtcaggtgacccctccattaaaagccagtgagatggatggagtgtgtgaattttaatatacacacaggcacatttacattacaaagcagcgaggaaaatctagctcctagagattaagcatttttgtttttgctttcatagtccccttttaccaattaagagaagctagtatagtataatgaaatgtaattaaacttttcagtgttaataacaaggctgtatcctttcagaatcatccagctgaacaattcttttaaacttgtaagcatgactgtttcttttcctttcaagggtcaaagaatcagtcattttactacttacacactttttcaaattggtcttttctttgacatccatttaaacttatcttgaagttaaggaccattgtaaaagacaataaaaataataatgtgaaaggaaaaaaaaataagtgacaaaaacaccaaagcacatagcataggtagaaatcaatagtttgctgttgtggaactagattcaataatgagtaatgctttgctctgagacaaataatttttcccttctctgtttcagtgtctctgtcttaaatagaaaataaatgtaataaatatagcaagtatcctcttcttgcaacccaatcaagcaagcctagtagagaagggtgtccagatgctaagaccacacagcaccccagagacagaaacaactggaaaaacttgtgctaacctagtatagtattgaagatacatttatagtctatggacctaggccctaaagagtaaatttgacaccatcttctcctctgctgcaaagtttttaatatccagtggagaccatctcttctatctctaccactgaatagaaaagatacgtaatctgctgttaggaatactgtaaagaaaaatgagataatatccactttctttcaagggtcaaagaatcagtcatttttttgaacactcagataaaaagtactttgtaaggctaggtgataaattattagaatgaagaccaacaagcatcagaagaaaactcttatttggcatttggtgttctgtccacggattcttaattcaggagcatgatgatactggtgcctcagcaaaagaggaaaatagaggaagagctgacatagaatcacattatccttgccacaaaagataacatttcaaactcttacacaaacagcctctccctccttccagaatgatgttggaagagtgttgcatttgctgctgggactgaggactgcagccgaaatacacccagtcccctccatcaacacctaaaatgaataagaactattcactgttcttgctggctttgtatttgcaaagctttaccttgcatggaaaagatcccatttaagcttttaaaataaattatatgctaactggctgcaaatttagcttcagtttgtgctacaaaaattggcaccaaaacattggacaataaaaaaatcttccctcgaaaagtaagtcggcttaggcaaatttagaaagacctaaaatgttataggaaaaaaacataaaagatttcactttatagcttctaataaccaaatctgctgttctttcaccttttcttttttccctctagcattggctgttttcattttgcatttattcagagttttgttttgtttgttttccctacttcacccactggcttttgttcttttggccatggagtcactttccttgaatgtgcaaaatgtaggcaaggacagacagtgagaaagacatattaccttagatcagataatttgtgagctttaaccctaacactagtgtattttctgagaagaccacaggcaggacagacacacctaagcatatccaatacagacacaactttcaggctccaagctattctaacagagacttgatgaacatggaatatggactgcatgtattttctattaaaaacagaaagatcatgacttaaagaagcctattaaaacttaccaaagacaggccagtcccaaaaaaaaaaagattgatataaattggcaaaaacagtatagcaactaaccctagccaacttttcaaaatgccttccattactcaaggaacaaactgaagtgctgacagagggtagaataaatgtttactaatgcactcatttattcaactaatgttcactgagcacttcttttgtgctaggcaccatactaagcactgaggggtacaagaaaaagaaaacagagtgtttttcagaaactcaaaacaggtacccattaacatgtaatagatgttggtacaaagtgctatggagtgtcagaaaaagaagaaaaattctccttaaggcgaggcaggacagtcacatagaataggtaaccctcgaactgagcctttaagtatgtgtcagttttctaggtaagtaaaggcagggggttttcaggcagagacacaaagaacacgaacaaacctaaagggctgcgagtgatcttaaatgttctgccaaggaatttgtgcttcatctgagatgtaatggcaagttatttaaagttctttggctagacaattacatgttttacaaagattattttagcagcaaggtgaagggcagatgacagcagtgttttccaaactttcctaattataagaattacctgcaagttatagtaaatatatatatcactgggttccactccaaatctagagaagtccaagaatatctatttttaagcagtatcccaggcaattattattatcataaaatttctggaaacactggttttgtagtgtttgctgagtaccagaatcacctgtagagattttaaccaatcaaatgcaggccacctctaaattacttgaatcagaacatctggggatagaaaccggaaacattgttgattttaatcttctaaggtggttccaatgcatccgaggttggtaatcattggtttggagagaggcaagacagaaaaaagactatttagaagctgttgtagaggatatttgggtgaaacaacagaattcaactagctcaagtaaaggagtactcgtgctacaaaaggcaatatcataaacataggaaacacagtaacgctgtacgaagcctcacaggaactggggctaagaagccactaaaaaccaagaatcctcttctctctctcagtggctgtataattcacttctttgattcttcctgtctcttatcctgaaccagctttcttttcttgcatgctgtcatctccagggccatgttgccttgtcagttctcatgtcagcaggcaaagactggattggttgggctgatttccttagtttgccactgatctcatcagttatagccagagtgtctcacattcactttgcaggagctctgggcaaagattttctgagaagaccacaggcaggatagacacacctaagcatatccaatacagacacaacagttcaagcaaaaaatgcttaagaagacttgagtaggctagtggtagaagagactaaaggtcccagatgcttttcagaggtggaactcacagaacatggtgactaattgaatatgagggtgtggaagagaaaaagtcaccgcagaagaataaatatattttcatttactgcagatgctacattataatacaaacaccactaagtgactatccattttactagtcagtagaggatatatatttggttttgaactccacacttacatatatatagaagcctaaaggtcagggccgggcgcagtggctcacacctgtaatcccagcactt

SEQ ID NO: 18950 - RNA, 8353 nt, Homo sapiens
  source 1..8353: mol_type = other RNA
tgcggggacaggccagggcatccctgaatgtcaagtatttgtttcacccgctgtcctgtaggactgtcggcaatagtgaagccgaagccctgggcacctttcacaatggttaaggtcataagttcagcttgggtggccccagatgaagccatagacacattgtcatcatggacgggcggtggatacgtgccgtctagctgaccatcagttggcatggagtgcagagaatgaggcggccgatctgttatatctggaactgactgtgaggtccgagaaatgtactccaaatatgtttcatagttgtgtcttccattgaccatcactggaggtggcctctccattattgcaaggggtggcaccatgctgttagcagggtcttcaggatcaaagggcaaagggtagccacgacacaacaccaggttgacactctgaccaataggaacagactggaaaagtttgacaacatctgcatgagtgtgtccaaggacacaaacttcattaatatagacaatgacatcacctgtttccatttttccatcctgtgctgcaggcccatccggaatcacacttttcacctgcagaaactcatcaggctcgtctccaccaatgatggtaaatccaaagcccatgttgctcttttttagggtggtgctgaggaatgttcccttcaactgggatgcatcccgggtgaagagtggtttttcgaacagccagggcctccctgctgggtcgcgctgatagtaagacaagtcattcacgctgcgcgacctctccggggcagcacgggggcggatggatttgggcctaggtaatgtccatgaggagctgtctactcggaaacctggggcctgcaggggctttgttccaagttctgtgtggggcatgttatgttgctgtagcttcctttttgcttccaggacaggattttcaaactgtgttcttctatttatgtggtcaacataataagtgccataaatgggatcatcgattttttcccagccatatggaagctcattttctttgcactcttctggaggtttagcctttttcgcaagtcgtggatccagccatgatgttgtctttgtgttatggtcaatgaagtagacttcgcccttctctgtataggccatttcccagttatcaggcaatgggtctggttcctcattgtcttcaggtttagttggctttgtgtcatccatctgctccttcagctcctcaggctgactgtacactggtgcaggataaggctgggagggcatctcccctgaggcacctgcacttttgtcttcatgttcactggattctggtgttactactactccatttccattgaccacaggcctctcttcctcttcctcctcaggaggctctatactggctttctccatgttgctcactgatttattcctcttccgttttccttcagcacttggagtggctcctggaagtatctggtctgttacatttaacaataatggtgctggttctgctggcggctttggggtaccgtagtaattgtcttcataagtcccactttctaggagagcaccacttttctccaattccataaaatcttcaacagtgatgaaaatataatccactccagggacctcaccctccttatgtggccttgtggtgcctcagttgtgtgatcaagtcagcatcaatactgataagccatgttgatagcatgtcttttggatctgatgtgatgaaaatgatgttttacttctatggacctttcttccccaacacacaattctaccctaaccatgaaacaaaacaaaaccaatcaaaacatcaaagaaatatcatctgagagacattctataaaatgcctaaccagtactcctccaaagtgcaagtcagcaaaaatctaaatatacatgatgactaaatgtaatatggtatcttggacaggatcctggaacagaaaaagaacattaagtaaaaactaaggaaatatgaataaagtgtggactttagttaatgttattgtatcaatattcgtccattaattatgattgatgtaccatatacttgtgatgtatgatgtaaataataaaagaaagtaggtgagtggtgtgtagaaactctctgtactatcttcgtaaattttctgtaaaactaaaattattctaaaataaaagatttattttttaaaaagtaatttcacacagccaagttgttataaacattctaaagtaatttctagtaacaatataaaattggttctttttaaaataagaattgatctgaccctttgaaacaaaagtatatcaggttcaaaaactgtctgtgcaactggagtaaattcactaactcttatgtcaactcagtaacattgaattcaaagggcaactgcataaatttaaaactttaaatttattaatctcaacaaagcttccttcatatttttgtgtattttgtgcagttacaagactgacatgatgtttttgatagcaattaaacctgcatattcaccttataaaaatgtacattatttgtatacattcatattatcaaaagcttcaatttgaatataaatttttattagtgtccatctaggttacaagatttttcttttctgtgaacttcaaatttatgttgtttatgtactttctgatactggtgagacaaggcaaaacatatgccttttttgtttttgtttatgaatatctggcaactatttctttttttcttgaaatttttgaattgaagttcatgatacagtaaatctttgtgaacctttttcatggctcaatcaaagattttttcatggctcaattaaagagcactggtaggatgcaaaatcagtatgtttattgtattctgtttctttgaacaattccataaactattgattattcatcaatttatatatgtatactaaatgattttaacaagtatatccctgacacttatcaaaaagcctgctatagataactcagtacaaatatttctggcatcatacagtgaaataaagccataagaaagacatcggtctcttgttttaaaattccaatctagagcatcaaccatcatgattgaaactactaaatttttcacatagagctgacattcttttttgacatttgaagattcaaaaatatatatccaaaagttcaattttttagttcacaaaattgatatttcttcataaattctgaagttctttttgagaagaatgtatccaaagtgttaactgggctatgtctctaatgttgtacgactcaactaaagctaaaaaataagcacttgtgatttttcaaattttggatttattgatatttggtgtttgttagaaagttcctatagactataggaaattgtttggtagcttgaattaaaatctttactttttgtaaaatatttcaaaatttgtttcttcataattttctattaacatttccataatcaaaataatttttcttttataactttcatcaaaatgggtttttgcttttggtgcaagattccaagcaattttatagcagttcaaagttacaagctcagaacttaaaaattatctaaaaatttttattggacatttaattcttacattgggcaactaacttcattgatcttttgctactgttgaaagaaaactatttatgaaaattcctatgtattttctgacaatgtctcttactcatgaccacttttttatctttaagaattgtttatacaacaaacagcttttccattttgctttgcttcaggaagtggtaattgccagtcatgattcattatgtaatatatcttatccaatctctttttttctttagtgttccccttgtagtactatcatctacatttccactccattctgcatccattctataattttgttttaaattttaaaatttgctcatattcacttttaaactagaaacacaatttaattgtattctggttaaaataatatgtattttagttttcctgtgattttcagttatctctaaaatcagggctgtctgcataaaatattcaaataaacacattacaatgaaaaaaaatgggagtgaggggtagcttggaacttagagtgtgattcaagaatgctaagtgaagaaaggattgccttctatgaggcagaaaagctcagaaaagggataaagagttaagggaatccctggattcctaagcaaaaaggggccaattggcaatctagctagccttgggctatggaaataagattcacacttcctcctgagacttgaatattacgtacacagcaaagtctcttgatatatgggatgaaggattcacccacatttcattgattttggggaagagtatggcagtctttagataaagggggactaagataggacatataaacttttcttctttttattagcataatgtacaatataacatttggttggaagtagaaacttgcatttcttatcaacattttttccccaaattcagagcaaggacataagtttggaagatatctcatcaatacaagcaaaactgtgatatgaagcccatacattatcagccacaccatagtttcattagtagattcatgccctattaggccccatccaatggctcatgtttttccactcttcaaaactcctccttccaagaataggttagatttccacatactattggtccctctgaatatgaaatgccttacatttttacaattttcatcctaaagattttcttctttgagtaagaatccaagtaattttacagcagttcagttataagctcagaactttaaaattatctttttttttttttgagacaaattctctctctgtcacccaggctggggtgcagtggcacaatctcagttcactgcagctcaagcaatctgcccaccttgtcctcccaaagtgcttggattacaggtgtaagcacccagccaaaaattattttaaaatgtttattagaggtttaattcttacatcaggcaactaacttcattgatcttgatttttcagaacaatgtaacagttactgatttgccccatttaacttctgtactttctacttctcccagcctccattgtttcaattagtatgttttaaaacattcacttcttttataaataaagttacatatcttttttcttctgaaaagttatatagtgaatttacatttcataccttcattgtacagcaagataaattgttctaattgatagaatgaggtcaagagagtaaaacactttaaacactctctgaaaagagagttataattttcatgtgaaatttatttatactggtggttattttcacaactgaactttaaaaggaagggtccatttggctgcatttgaattggtgacatttttaggctgtcattacctgcagaaagagcgaatcagtgtgtcaatatgaatgagtggtaagtgaccttttaaaatgtttttcagaataagggtttctttctttctcttgctattttttttaaataaaatatatctgaattagaaacatgatgaaccctaactaaagctgctcaaagtattctctgaagaaaaaaaaaagccaattattttctcttaaatattccttacagatagaaattctaagaattggtagttaaaatgtaaattatatttctgttttttgactactaagaaaggaaaataatactaatttttttttcattttgtattcaactaatattcattgaatacatgacatgtctaccatgcagtttttaaagtagggttggaaatacatgaatacataaaatccaatcctcctttataaggaaattttattttattggcggtgacaaaatgcatgaaaataattcagtacatagtaattgtaagggcgggtggaaataaaatagtttagggggccatctttcatttgtcccagcagatacactatgccattcttcacgctactctgttttcctgaaaatctggcccatatgaatgccagttataagcttcggcttctgttgagtttgaccgtcagggaggacctgcataatctcatgatacaagggggaactagaagagtaaaatgtaaggagacccctgaaactattgctacggaataaaagatgaaatgctcctgattattgtaaatacaaagtggcatgcaggattgtgtaaagacaatgccaggttggactgccagaacgagccaacagcatgtgatgtgcttccccctgcagagagcctatgaatggacgtgcagtcaggggggtttcacatcaccaagattcctatcccagaaaggcagatgttcatagctctgggaatggaatgtgacccttgtggagagcctataaaccgacgcatgaggggcacctgttcatatgtataagatagggctataaatgccctcatcttgccacggctcttctaggcctctttagggttaaggcatactgccttctgagaatttctggtctaaccggttgtctagcttcacatcatgtttctatggattgtttgtaaccagcttttgctacaactgttactgctgattaatatcttactaatcataggttatggaaagactgtgtttctgttttaaggctctgttagaaattactgatgcacacactatattgtaaattcttatctctgtatactgtacttctgcatacagatgttacattaaagaattacttcatccccatgtgaccatctcacctcataatcaaatgaccctaaatccctcactaaactatccctgccctcactaaacttaataataaatgctggtatatccagtgcattggaggcatcaagggaccagaaggcagtgacccccctggactcagctttcactatcttgtgtgtgtctattatttctcgacctgccaatctgcctgggaacaaagaaagagccccgctgtattgcgggctgttggccggatcctgcaacagtaaagttggagtacttaggggtatttagtctcctagctccctgcctttgacggcaaagtgggcttgggtgtgtccctgaaccaaaaggctcaatgcctgaccaggtgtctcctcacacagccctctctgttcatatcctcctaacttaactcttccattgttctctaaagcctaggggcttcagaagcagcgctgaagcaccccagggttctgtaatatcctttgttgttgtactataccctgcctaatatacaaatgggagagtgctacctgcttcctatccagtctgaaatggaagtttttgagaacaaagtgatcacttctagctgttaggaacaattttgttatctttgattatgtagtatataatggttagaatagaaaactgaaagttttttctatactccatagccagaaatcattttactaacgtgaaagtcattattatgtcccctatactttaaaattcagtttttggagatggagtctcactcttttgcccaagctagagtgcagtggtgtaatcatagctcattgcagccttgaactcttgtatatcccttattttaaacaaaaatttgaatattaaatttacagttctctggacaatatgggcatggcttcaactctatttttatcagagctttaaaaaacttgagatgtatttcatgtactgcaaaatttacccttttaaagtgtacaggtcagtgatttttaatatatttcacaagtttgggttaccataaccactatccaatttcagaacatcttcaccccgcaaaaagaaaccccacatttcttagccttctctctccaatcccgcatcctccttagttctatgcaactactaagccactttctgcctctatagagctacctttcctataaattttctataactgaaatcatatgatatgtggcttctttcacttagtgaaatgttttcaagttcatccatgtcatagcatgtatcagtttttcattcctttttattgccaaataatatttcattgtataaatataccatattgtatttattatcagttgatgcatttaggttgcttccactgtttgtccattttgagtaattctgcaaatgaacacatgcataaaagctttatgtataatgcttttgtttgtcttagatattgatatagtttgggtatttgtccccacccaaattgcatattgaaatgtaatccgcaatgttggaagtaggtcctggtgggaggtgttttggtcatggggtggatcccttatggcttggtgctgtacttgcaataatgaatgagtactcacgagatctgattgtgtaaaactgtgtagcacctcccctccccttgctcctgctttcaccgtgtgagatgcctgctccacttcaccttctggcatgcctgaaagctccctgaggcctcctcagaagctgagcagatgccagcaccatgcttgtacagcctgcagactgtgag

SEQ ID NO: 18951 - RNA, 17408 nt, Homo sapiens
  source 1..17408: mol_type = other RNA
tgcggggacaggccagggcatccctgaatgtcaagtatttgtttcacccgctgtcctgtaggactgtcggcaatagtgaagccgaagccctgggcacctttcacaatggttaaggtcataagttcagcttgggtggccccagatgaagccatagacacattgtcatcatggacgggcggtggatacgtgccgtctagctgaccatcagttggcatggagtgcagagaatgaggcggccgatctgttatatctggaactgactgtgaggtccgagaaatgtactccaaatatgtttcatagttgtgtcttccattgaccatcactggaggtggcctctccattattgcaaggggtggcaccatgctgttagcagggtcttcaggatcaaagggcaaagggtagccacgacacaacaccaggttgacactctgaccaataggaacagactggaaaagtttgacaacatctgcatgagtgtgtccaaggacacaaacttcattaatatagacaatgacatcacctgtttccatttttccatcctgtgctgcaggcccatccggaatcacacttttcacctgcagaaactcatcaggctcgtctccaccaatgatggtaaatccaaagcccatgttgctcttttttagggtggtgctgaggaatgttcccttcaactgggatgcatcccgggtgaagagtggtttttcgaacagccagggcctccctgctgggtcgcgctgatagtaagacaagtcattcacgctgcgcgacctctccggggcagcacgggggcggatggatttgggcctaggtaatgtccatgaggagctgtctactcggaaacctggggcctgcaggggctttgttccaagttctgtgtggggcatgttatgttgctgtagcttcctttttgcttccaggacaggattttcaaactgtgttcttctatttatgtggtcaacataataagtgccataaatgggatcatcgattttttcccagccatatggaagctcattttctttgcactcttctggaggtttagcctttttcgcaagtcgtggatccagccatgatgttgtctttgtgttatggtcaatgaagtagacttcgcccttctctgtataggccatttcccagttatcaggcaatgggtctggttcctcattgtcttcaggtttagttggctttgtgtcatccatctgctccttcagctcctcaggctgactgtacactggtgcaggataaggctgggagggcatctcccctgaggcacctgcacttttgtcttcatgttcactggattctggtgttactactactccatttccattgaccacaggcctctcttcctcttcctcctcaggaggctctatactggctttctccatgttgctcactgatttattcctcttccgttttccttcagcacttggagtggctcctggaagtatctggtctgttacatttaacaataatggtgctggttctgctggcggctttggggtaccgtagtaattgtcttcataagtcccactttctaggagagcaccacttttctccaattccataaaatcttcaacagtgatgaaaatataatccactccagggacctcaccctccttatgtggccttgtggtgcctgtgatttcatctttggtaggaagctttcttagacatctctggcctaggtcagttgtctggcctgtgtttcaccgttagagcattcatcatacttttcccatgtctgtggccatcacttcagttcacgtttattttgtgactatactgagcaccatataagctagaacacacagtacaaattacatttactatcccagtcctcaatgagtttcttaggagcttagttgaaataggccctgaagatggcttgccatccggcagaatttatatgtgtttgtgccttagctaattcctcatttctcatcttcagctgctgtcctcagctatatctcttagtatcttctatgcttggctcctggcatttacacatgatcttttggtattgactttttgcctggtctatgtttgtaggatcacagattaaatactctgctccctcataacttcccagtatttaccctgtacagcatgtttctcttgtgtcaatcctacagccagccaggtcagcacagtcttttcatgactcttcttttagatcacaaacctagaagtcatcaaaccttcaaacagaactttctaagttactaacatatccaggagggtaaatgcagccctcaacagggaagggacctttcacgagagttgcctcatgttaaataagcattgctaacagaatggttatttctgttaataagtacatattaccacatactaagtacatattacattatttaatccttatagcagacaagattacacacattctactaaacaggaagctgaaattcagataagttagtacctagtccaaattcacacagctagataaccatcaaaatcaggactaatgctaattttaaatcctttgccagccctgcatgatcctgattgagtccaagtaccctggggattcccaggtcttagcataggtggtgcaaagaaccctatgtttggggagagggtgtaggtaatggataccaaatcactccatattaaccccatcaaagaatgtgactcttgacccattcttagagaagtgaactacaacataacaaggaggaagcaagcttaatctctgaatgaatctggagttttatctgtccatggcacgataataccaaacacattcctcagggggctattgcaagggtgggtacaatatcctattgatgaaccgtagtgatcaaaggaaggcatgagttgagagcttaacagagagaaatgctcataaagctcagtatattgctactgatggaatgattaaatgccgcttgacacaaaaacatatgcagttcttgaaagtcaaaagatacaaaaactctagagtcatatggtttgtcaatctacaggcaacccctctgtacctataatttcacagtttcatttatgctttgcaaaattgatgattattaccaaaggaatttgagtttaagcctggcaactaaatcaaaaagtaatgctcttaccatctagaaaatacttaaacaactttaaaatggagtcaatgaatgtttgactgtttgacaggtaagctctgagtatataattaatctggcaattgaaatcagctaagtctttataaattctctttgtagtctagtgcatgatgatcacaacatcacttgtaaggactttgcaatattcaaaggactgaggttcatactcacatttagtgatatgaagttcacaggatatatgtgtgttaaacttgcacatcattgaagtttacgtatataattaattagactcaacaaaggaaacattcattgtctatttgaggtctggactgtgctggcatcagcatgagccccctactaggtctcagactaaagaggtgtcaaagacaagcaaatagtttcagaagagtatatataatagtaataataaggtaacattagaaatatgagcaaggaatggaggttgcagagaggagggatgttattacctagaaagggtgatttcataacgcttatgtgtaaaatgggggcaggaataaaatgggtgaattagatcatctttatagtctgcttttgctctctaattttgtcctgtctatatacttgtcagattatttccattttgttcttttttccccttagagccatattttctgattatgaccattggaaatgttatgttcaaaaatttccatgatcaaggactgacgatggagtctttaggtccccagcttctcttcttacctccttcctaagagctttgtaggatactgttgctctggcatatcttctccagagactgagtagagaaaggaggtggaattacaatcagtcagcttcacttactgaagttcttgtgaaagtttgatagaagagagcgttgatgtttaagaaaatatttttcacagaataaggcagctcttaattacctgcagtaatggagagcagtggtgtgtataatccaaaatggtggataatccaaaaactatttctatttgactttgaaatgtatttttgaacttgcatttgaatagaaatatggcaccaacaacttaaagagtcctaagctttctatctttcttatacacattggtctttagaaattgcatgtttgagttttaagaccttcctccactggactgcaggtcaactctaggttaaaaggaacagtgctactggcaatgtcaacaaaaatagctaagcaagacatttctaaaaagaaattaaaataaaatgtatcttagatgatgtagagtttggctacatattgcttgattatatacactcgtctatgaaccaagttcctacttacagtaaatcatttaagctggatgtgatgcacatcatttcaagctgatggaaagatgactagataaagtttgttctgtctgactcccccactgaatgcctgcctggcactctgaggaagccacagcagggtgtcttcagaagctatttccaaacaaatttagacttgtcttatacatgatgagagctatttataaagattgtataacaaatagcttataaaagacacctctgtcaattgcatttataatgaaaaaatctaacacaagaaggcgttgattcccagtgcaagctaacgctgcagtatctttgcttttttatcagctaaactaaccggggaaagggagcatgacaaaactcactgcacttcattgaaacttgaattgagatcttaaaaagaagtagagtttcatcaaaatatacaaaagagtaaagggcagtaggtgcattttagttggtaaagtcagaatccagcaatcatatcgaatgacaagatctactctcagaaatgataggtaatgacattattatgtgaggatctttaataacttctactgttatctgtttaattgatgtacaaaaggcaaaaagatttaaagaattgagagaaaagcagaagaaaacatcaaaaatcgaagaatttaaatcttccatccccaagacaaatggaaagcaaaaatcaatacattacaaaaaaactaaataattttagtgtgaatgttttgaaactatcagccatctgtagtaattgtacaggcaaagattttagcatcgcaacaatctaagatgggaatttacatacgaaaatgaaaacattagacctttaatcagaagaattgaaatgaaaaccaaaattacttaatattttttccccaaaaaatatgcttttggaaatgtgagactatgtttgaaagcctgtgattttcttattttataaacgtgaaatgtgttcagtgatgactatgacatgacaatttggaaccttgaatttagtctcctattttactcctaatttgtaatgttaccttgtgcataatgtttattcctttggggtaaagtgctaattaaataattcattcattttaataagcatttcttgtgtacttatgtactaggccctatgcttggcataggagctataaaattgaataggccctggttatagttttggcatatttgataaagtcagtggggatgaaggcagaaagacaaacatgtggcgtaagatggcactttgactaaaactacatacaagtggagatggcactaacagaaagtgaccatttctacatgggatgagatatatcaaggaattcattgacagactcagtcttacagaatctctatacatcaaaggtatttgccaactatccctcttctgaaaggtcaagaagtcaaaatccccatgaaaccttgaatggcggtacattaaaaaacaagaaccttcaaaatatgtaatagctcttttcagagctgtcatacacaaataaatacaaaatctactcttacttgctttccttcaatagtatcacaaaaggaggtactatgttgattcagtatatagtttgtatactcacaatgcatggaaaaatgcatggagaaccatgcatacagaacgttttacctcacgtattctcaattgattttctaacttttgtttttagcaaccatccttcatcaaaaagatccaagtgttaaataaacaagtctagaattcacagtttgtactctccttgtgcttcctcgttttctgttatttcttttcggcttgggtaagcaaactctgttactgccacattcttttttttttccactgagaatagtttcccatgttttcaaaagagcacagttgtgtgatatgtgttgtggggggaagaggtgaaagaaagaggggggaagagaatatacttgtgtaaatatgaatagtgtacataaacatatatgaagacatggtcttctagacacagaagaaaaaagatacataaatgaacacaaagtgtggaaacacatgtgtagtcagatggatcagtgtccttagggggcaaggtttcaaagctcagtctacaaaaccattctaattaaaataacattttaatatccaattctgctttactttgtaagcattttctcccttctgtttgttttctttactaaagtcacagcaagggctgtgctgagcctccagttcatctaagctactcggtgcatgcccagacagcaagaaaatggtttctctggcaacaggaattatgtgaaatctctgtgtgttctcccccaccttccatctgattcctattcacttaagctcttcacatataggcaacaacgaggcattggaaatctaatgagcaattcaaatttattgagctagttcatggaggcgggtactgtgagcatcttcatttcctgtgtaccagggagcagagtgtgtttgttgtacgttatctgtattattcaagaaccatgcactgtcagcaaatagcccaaaccagataaaatcagatgaatatctaaaataagaagcatatgaggaatttacttccatcatggtaggagggaaatgcaaaggctttcaggtgccaaacacagctttgaattttccaaagatgctgagcgatggaagtcacaatgatttaaaacagcctcatattgtgtctgaaacccaagagggaatggcaagagctttgattaaattgctttgaatgtcagcttttttatttctaaggaatcatactgttcctccatgactaaagcgctagagttttcaatttaggccttataaacattccctaataatagttcatgatgagacctcttatatatgtttttctctgtagcctttgttaaggagagagtcctgtgtttagcattggcactaaggctgatatttactaagagagtttaatcaaatgggaattgatttgcttggaggaatcaggactaaggcaaattagctttattctttagagattgggagaatgtgggagggaaggatctatttttcttcggttccagtaaggatgaaataacagcaagaaatatactcagtaacataaagtagaaaatagagtgaattggaatggactcctgaaccggtttcagaatcattgtcctggaagtttaagaagaatatttgcttcttactgtctagaatattttagtaaactctacctgcaaggaggtatatttttaaagtttccttggttttatcattgtatatcttacctgttaaaaattaaggactttgtcaccaaaaagcaataggaaatgcctctttgcataaatctttaatctcaatctacatgatatagatttaagtaataactcaatgaaagcccaatttaaataaactttaacttccagtgaaagctgtaagaaagcaatgagcagaatgattagcctaatgacacaaatatagtaaatgattaactaaaaagcatagaagggtgaagataccaaagacagatgacagtaaaataatagtagcattataacaatgacttcattcatttcatggttaatctttagataataagaacatattgttttagataataagatagtttaaaaattctcaaataactggcatttttcctgggatataaaagtgccaataagtacagccaaaatttggaaaataaatacaaaatataagtcctacacagaagagacacctactgaagccataacactcggaattttcaatccagtcacagagcttttaggaaaagaacatcttggaatcataatttcattccagttagaaaatggagattcaacactcatacctaaaaccaaattgcccttcacgtggtaagtcagataagctgagactaggggctttgtgtatgtagctagtgcttgcttctgggaacagagaaattgttcctgtgtttctaaatgtggtaccccactgcaagtagtgtgtagtagaacgcataaagatttactgaagttttcaaggaatttctaagctctggtctgcagttcttttcccacagagccacctttcaattgtgacttttgctatgttttattttaattttatttaattttaccctttcttccaggaaaagttgagatggcttactattatagtgtatgcatgtatcaatccttgaaaacagtatttcttttaaagagaaaattgcctagaatcaggaaaatatcttgataaggcacttatggtagaaagcagaagatgagaacatgtgttagtaggagagaaagcaatgaaaaatagcaaaactgttcctaagttagaaattaatggcaattagtgggtggtggggaatacaaaaaagaagaaaggaaaggcagagtggcctttagagggaaaacattaaaaattttagacatctaatattcaattttatgttgttgctgtttttacaaaatctttctcataattcagaaaagtgtggtacattcacattgctgagcacgctgatttttatggaaatgtgtttatcatgtgtgcttaagaaagatcaatttccccatttggctatataccagagcagggacacagagtaaaaaacaaaaaagttgtagagaaaagtggttcaagacagaggtgtttatgaggatgtaagacccactggaagttcagagaaaactgaagaactatattgggcttttcatggggcacggaatccaatcttatttacagcttaaaaggtaagaggacctcaggtaactgttagcccaagccacagcattttgcagactcccaccttttataaactccggtcagagtggaaaattccaccagagactgaaccgtgaagaaacatcttgtgggacaggtcccaggcctaacccctaacccagtgaattccttccttatcagcagcccagcataccattcccaccccatttcacagcaacctcagacctctcccgcctggacctacaactgccccagcctgcaagcgggaaaggaggctcctgcgctcgctggtgctccccctccgcaggtctttgtccaataaacctgtgttaccgtcgagccgccctccttgtctttttttctccatcttaacagtaacatggaagttataccacacaacacagcacacacacacacacagagtgaaaaggtaaaacgttacaatttttaaaatcagaaacaggaaaggtatataattaagcaggatgcaacatctgggagaagaaaaatgccatatatcaatgaactgtgtacacttgggcaatgtaacattagtgggccagcttcaggaccttactatggtgaaaatctgctacaaatttccactctctttgaagtcacatggatgtgaatcgtgtgtgctttcaacgtactagctgtgaatgaacttaggctagagggtgaaaatatcggagccccaatattctcctttcctgtaaaatacagatagtagtatctactttaaacataaataataatggcaaatttttatttactgcaaactatatgtcaagctccaaacttacagctattatttatttagtttactccttgcaactattctttgaagtattattattttcattgtacaaatcaggaacctaagcctaatagaaattaaataactttcctaagcacagagcttgtaggtagtggagccattagagtggttcactagtactgacaatagcagtactagtataagtattagtactagcataagtactaatataagcaaatactgtgaaagtcagtttcaacttgaaattttcaattactgacttcgttttctacaatgggcaaacccaagataactctgtaatgatggatcctttgtaaactttacttcttgtcattctgcatttttttcactatttctttatttaacaagggtggaacgccttgctcatttatcatcatagctgaattcttattagagcaccagctaattcatgcttattaagtagaaaagcaatggcaactaggcttgatgcctaagtaggattcaagcctgtatctaaagtgacaaaaaacttataacgctgtttcagatcaactatagagtggcaggaataaataccattgtatatgctcactgtaaagctagattatgtttccagtgtagtcacaccaagtaggagcacataccgtccatctcagcactttgtcctctagaccaggggtcctcaacccctgggccatggactggtaccatcctattaagaactgggccacacggcagaggtgagtggcaggtgagtgagcaaagcgtcatctgtatttatagctactccccattccttggattaccgcctgaactctgcctgtcagatcagtggcagcattagactctcatagaagcaggaaccctatcttgaacagtgaatgtgaggggtgtaggttgtccgctccttatgagaatctaatgcctgatgatgtgtcactgtcccccatcacccccagatgggaccatctagttgcaggaaaacaagctcagggctccccttgattctatggtgcattgtgtaattatttcattatatattacagtgtaataataatagaaataaagtacccaataaatgtagtgtgcttgaatcatcccgaaactatccatccccgcacccccaacccctgtccgtggaaaaattgtcttccatgaaaccagtccctggtgcccaaaaggttagggaccactgctctagatgattcactggggacatacggttgccagtgacactgtagggtcttaccaggtctggtaaacccaacctttgttatgtcactgtgcttttatacttttcacttacatcaccatttggaaaagtgtagactaacaatacaatgagggtttgtgtgtatgtattgaataacagacttggcattagaaatgttgcatccttatgtctgtggggaaaataggatgaatatctagatttacctgaagaatttctctgcctccagctttccaacattctggagagccagtttccctataccttctatgtgaaccaattaataggatgttaaagaaaaaggtaagaatttgtttgaactcaaggatctgacacatgctgttccaatcaattttacattctaataaaataaacaattgaagtcttacaaatactgcatgtccaaataaaataatacccattttttgtataataaactaaagcttatcaaatagcttcccttaaggttgaaggaaaaaaaataaagaaaaaaaatccaactgtaagtgaccttcaaataacctaagcattgtgttggcaagtttagtaagactatgttctccaaaagtttacagaagtgacattgtcatcagtatgtctactgaaaaaggagtgagtgatagaaaccactacgtttaaaaaaatcatttagttagaattatgatcgtgtattggggtttatgcaggatcttgcacgaagaaaataagcaagttgcaaccctctttcttttactttcaacgacaaaggtcatgccaagggtttggaatcctattgctgctattaagagctctttctatgcattaaacttgtctcaccaaagcaggtgtttgacatatgaggggcctggctgcagtactatcaatagtttcattacaggggacttactctccaaacatacctttcctgtggacagaatttaatttgaaccatcttttctagagggtagttgtttgtgattattttcttgaaataagtaaaaagtttaaatagaggtgatatgcaactccagtttaatgtgtgcactaatctttcactttatataatttatcatctataattttagttattataaatatttagttaaatctactcggttatctttcattaactatgaactcataatctacaaaaatatatcaaatggctgcatttccacattttccagaatcatatatcatagtactgtggctagataagattacctaaaatgcagataaattcttttgtaaatatgtcaaaatatatctaattaactatatataaaattacaaataaatcctgccttcctaagagggataaatttagaagcaacatttggagaaacacagtactgacatctgataagtatgactttgtttttcccctaagctataaatagtaatagctaacactgaatgcttcctatgtgccagtcatacaacactgagtgtgtactaactcacttaatccttataatacacctatgagattcaaactattagggatctcatcttatggatgaagaaactgaggtacagaataattaacttgctcctagacacagctagtaagtgaagctgacatttaaatctggacagtatgggtctaaaatcagtcatcttaaccattagttgtataatttatttagatatataatttataatttataaaatattattcattacatgtcagaataatctcttacatttaataatgaagaccacgagaaatggtccatttgtggtacaggacaccaccatatacaaagcagcttactaatgtacagctgtcgtgggaaaagatgtttctaaatcatttgtaccctggggacactacatgccattttattcaaagtccatggagattaatttctcaaaggataagttgagaaaaaatcatcttttccttcatcagaaaaccaaataatcaacttttatttctcaaaggtaagaaagatcaaatagacaacccttggatctaacctgtggttccacaaaggatataaaaatagcaagtgtgatgaatggatcataaaattgttccttctggggaaattctgtgatttaatgccacacagtatgtaaggagaatcgcaacataattgattgaaatctgaaatggagatacagggggcctaatcatttttctagaagaactctgaagaaagagttggacctaacgtttaaaaagctaacatctaacattaactctagtaagcaattataccagtgcttaaaccaatattacataaccaagaaaaaaataggaaatctatgtattctgtttacatttttactcacccacactgtaccagttcttcctcatggctgggtcctctctaataaatggaatttttgtataacatcttttaggtcacctaagcagtgatgtataaaatcactgtatatgtatgtatatgcccagaatgtatatgcccagaaaaataatgaagtctctcagcatatagttagctatcacagagtgactaaggtagcataagaattaatctcaaataatcctactatttgtaggttcctttaaaaaaatcaatatgcctgtaccttcaagttaccaagggcatatgtatgacatatgtgggttacctgatactttagaaagcagagaatagatatccccttatcacagaggcaggtcccgggtagatgcagaattttgaaaggaacatattgaaatcttctaatttgtgcttatcttgaaattaaattcagtcttctagtcattccaattttttccaacctattaaattgtgagaaatctgcaaagaatttattgagaaggttctcaaagaactaagatggtagctttttactaagaaactgattatatcaaggctgaagggtaagatttgttcagacaagctttcctagctagcatccaatgagtattagaatttccaagtctaatttataaacccaaacataaacagataaaaataataatttttattttcttcaagagaagagaaaaatgtaaggtagagtgaagtaacatttagactcagaaaatttaaatcaaagaactgacataaacaactagcaaacttgattgtttagattttaataaaatgtattgtataatctattattacttttagtgagagcaaaatattatagaaaaacttttttatttgtaaaatatatcttgttccaaggaaataagtatacgtaattaactaacacccataaaaggtatgactctttaatgttgtcaatgaagatttaacataatattctataacaaatatagctcattctgctcttaaaacacataattcattacctcatttgaatgtattgtttaatctaggaaattgtataataaatagcagtaataatatgggaataagcaatgtagttttactttcaaaactaatatccaccagtaaaactaaaatttgaactgtgagaaggcgatatatctaatcatgacactctcaggaggaaatagcacaacaattttaacccattatttgtcatatttctgcatgggaacatgtttcaaaataggtttcataggcctaacacataacccaggaataatcgcacaagtaattttgagggtatattcatagtcacctttccatattcaaatgttacaaaatgaatttctaccaaagacactattttcattcttattagagttatttgctcaagactatagccaaagaaatatagatcttaaatctcatcatcaaaaaagcccagaactctggcttcattttcaggcacaataccacaatggcaaaacatcagtctcagtgtgatatatcagttaataacgtaagcagtaagacacgggctaaatttaacacatactcaaaacaacctctgttaaataatttaacatgaatgatattaaggacaattaaatacatttgtttcttagacagtttgtctaagagtcttgaactcttttgtgagaatccctgggggaacttaaatgtgggtacttatgttttataggattgaccaggaatagtctaaaatcagaagtcatagccctcctaaagccatatagcttaattatagaataatataatcatagaattatagttggcttatctagttgatgcgattcatattaaaggaaaaggaagatgtaagaatgtggaaattattgccaaagagcactcagtaaagttgctaagagaaaatggttagtaaatcccaggccaccttaagatattaagttgtctgttaagcattgcagtgatcaaggaagcatccatacttagaaacgcatgattaatcttttaaataatatcctaatattgtttaaatatactttgatttttcttcaaaacaaaagaaaaatgtaaactgttattttctttggtcaatatatatgtttataagatggccttataaattctattgctcattggatgctggctaataaaatacattcatccattttctttcaatcaaccatatttatttagcacttactaaattcaagaaggcctgggccctaacacatttgtaagtgtgggcagaggcctaggaatttgcatatttaataagaaccataagtgattctgaaacaagtaagcttctgaccaaatattgcaaaacattgataagggactgcttcaagggggagaggcaatgacaacatcatgaaggatgcagtatttgaggtatttctagaaaaataggtaaaattagggtatgtagagatagtatgaagggcaattaagaagaggaaagagactaagttaggcacaagagcaagagggtgtagagtgaggaaataaccagtggcctagattggctaacaataagaaaattagagagtaacagaagagatgactataggtcagagggaaattgatttggatcaggaatgtcaaaaccagggagtactgactctattaaatacatgacagggagtttctaaaatttcttgagcaggtaaaagcttaattcaaagtatagggagatagatgttgtgaaaggtagttgaagccatgggaggaggtaaggttgctggggaggcaaaacagaacatgacgaagccacactcgggaataacattgaggagtgtctacatttgattgcctggagaaagaggaaaaaagaaggaaaactgggtgataatgttaccaaaatagcaggggtgtggtctaggtcctgctgcttgctgcacagaaagtcaatcactgagacaatgagtactgccagggaagaaggctttaattgggtgctgtagctgaggagatgagagatcacaatgaaatgattaaaaggataactaaaggaaatgtatagaagaatgaaaaggttgagtcaggggcacagcatagtaacatgtaggaagagaggatatagacattacattgcctggggacatctctttccctctctaggccactagcataggttcaaaacagagactaaattgcaatgcttatattctgtgtagactaaagactgaaaaagtaatggagctttactaaaagatgggtttcaaatgagagagtcagatgaaagtgcaagggatttccagcacctatgatggtaccatagttgtagatggcaggaaagcaaggagcagaagctttcaagtcgagtgcacagtcattttaaaaatgagaaggtgcaggaaattgatgagggagtttacagaacccaactgtctcacaatttgcattaaagtatgggcgcccttatttagtttgtggagttctctattctggcccttagttctattgctcctgttgaggaggaaggagaagaaaggttgcctgctcctgtgtgcctctttgaggtgccaggagattactctgaaatgctttcctagcatgtagcatgtcttgtacagcaattccagcactgagacatgtaccctgagatatgccaacacacttccagctggtccaaggctagaccacctaacttttgagtttcaacttctaataacaatgcataacagcacttgccagttgcaccattttacttcagaaggatgtcacatgaatcattgaaggagtgactttagaagaccttgagccaattggagagaagcgctctaagtgcccaataatttctcatttttaatattcagtgaagatttttgaaatgttaaagaaaaaaatagaggaactaggaataacaaatggctagcaggacacatttactggaatgaaggaggattgcaaagctattttctcaattatattttttacattaaaacaacgttgcatttttaagccctgcagataaaatgtcttttatgaagaaaagctaattaagtttcctgaaaaataaggcagctggttaacaatttacgtcttttttgaagcgttaacgctt

SEQ ID NO: 18952 - RNA, 15723 nt, Homo sapiens
  source 1..15723: mol_type = other RNA
tgcggggacaggccagggcatccctgaatgtcaagtatttgtttcacccgctgtcctgtaggactgtcggcaatagtgaagccgaagccctgggcacctttcacaatggttaaggtcataagttcagcttgggtggccccagatgaagccatagacacattgtcatcatggacgggcggtggatacgtgccgtctagctgaccatcagttggcatggagtgcagagaatgaggcggccgatctgttatatctggaactgactgtgaggtccgagaaatgtactccaaatatgtttcatagttgtgtcttccattgaccatcactggaggtggcctctccattattgcaaggggtggcaccatgctgttagcagggtcttcaggatcaaagggcaaagggtagccacgacacaacaccaggttgacactctgaccaataggaacagactggaaaagtttgacaacatctgcatgagtgtgtccaaggacacaaacttcattaatatagacaatgacatcacctgtttccatttttccatcctgtgctgcaggcccatccggaatcacacttttcacctgcagaaactcatcaggctcgtctccaccaatgatggtaaatccaaagcccatgttgctcttttttagggtggtgctgaggaatgttcccttcaactgggatgcatcccgggtgaagagtggtttttcgaacagccagggcctccctgctgggtcgcgctgatagtaagacaagtcattcacgctgcgcgacctctccggggcagcacgggggcggatggatttgggcctaggtaatgtccatgaggagctgtctactcggaaacctggggcctgcaggggctttgttccaagttctgtgtggggcatgttatgttgctgtagcttcctttttgcttccaggacaggattttcaaactgtgttcttctatttatgtggtcaacataataagtgccataaatgggatcatcgattttttcccagccatatggaagctcattttctttgcactcttctggaggtttagcctttttcgcaagtcgtggatccagccatgatgttgtctttgtgttatggtcaatgaagtagacttcgcccttctctgtataggccatttcccagttatcaggcaatgggtctggttcctcattgtcttcaggtttagttggctttgtgtcatccatctgctccttcagctcctcaggctgactgtacactggtgcaggataaggctgggagggcatctcccctgaggcacctgcacttttgtcttcatgttcactggattctggtgttactactactccatttccattgaccacaggcctctcttcctcttcctcctcaggaggctctatactggctttctccatgttgctcactgatttattcctcttccgttttccttcagcacttggagtggctcctggaagtatctggtctgttacatttaacaataatggtgctggttctgctggcggctttggggtaccgtagtaattgtcttcataagtcccactttctaggagagcaccacttttctccaattccataaaatcttcaacagtgatgaaaatataatccactccagggacctcaccctccttatgtggccttgtggtgcctgtgatttcatctttggtaggaagctttcttagacatctctggcctaggtcagttgtctggcctgtgtttcaccgttagagcattcatcatacttttcccatgtctgtggccatcacttcagttcacgtttattttgtgactatactgagcaccatataagctccttcctaagagctttgtaggatactgttgctctggcatatcttctccagagactgagtagagaaaggaggtggaattacaatcagtcagcttcacttactgaagttcttgtgaaagtttgatagaagagagcgttgatgtttaagaaaatatttttcacagaataaggcagctcttaattacctgcagtaatggagagcagtggtgtgtataatccaaaatggtggataatccaaaaactatttctatttgactttgaaatgtatttttgaacttgcatttgaatagaaatatggcaccaacaacttaaagagtcctaagctttctatctttcttatacacattggtctttagaaattgcatgtttgagttttaagaccttcctccactggactgcaggtcaactctaggttaaaaggaacagtgctactggcaatgtcaacaaaaatagctaagcaagacatttctaaaaagaaattaaaataaaatgtatcttagatgatgtagagtttggctacatattgcttgattatatacactcgtctatgaaccaagttcctacttacagtaaatcatttaagctggatgtgatgcacatcatttcaagctgatggaaagatgactagataaagtttgttctgtctgactcccccactgaatgcctgcctggcactctgaggaagccacagcagggtgtcttcagaagctatttccaaacaaatttagacttgtcttatacatgatgagagctatttataaagattgtataacaaatagcttataaaagacacctctgtcaattgcatttataatgaaaaaatctaacacaagaaggcgttgattcccagtgcaagctaacgctgcagtatctttgcttttttatcagctaaactaaccggggaaagggagcatgacaaaactcactgcacttcattgaaacttgaattgagatcttaaaaagaagtagagtttcatcaaaatatacaaaagagtaaagggcagtaggtgcattttagttggtaaagtcagaatccagcaatcatatcgaatgacaagatctactctcagaaatgataggtaatgacattattatgtgaggatctttaataacttctactgttatctgtttaattgatgtacaaaaggcaaaaagatttaaagaattgagagaaaagcagaagaaaacatcaaaaatcgaagaatttaaatcttccatccccaagacaaatggaaagcaaaaatcaatacattacaaaaaaactaaataattttagtgtgaatgttttgaaactatcagccatctgtagtaattgtacaggcaaagattttagcatcgcaacaatctaagatgggaatttacatacgaaaatgaaaacattagacctttaatcagaagaattgaaatgaaaaccaaaattacttaatattttttccccaaaaaatatgcttttggaaatgtgagactatgtttgaaagcctgtgattttcttattttataaacgtgaaatgtgttcagtgatgactatgacatgacaatttggaaccttgaatttagtctcctattttactcctaatttgtaatgttaccttgtgcataatgtttattcctttggggtaaagtgctaattaaataattcattcattttaataagcatttcttgtgtacttatgtactaggccctatgcttggcataggagctataaaattgaataggccctggttatagttttggcatatttgataaagtcagtggggatgaaggcagaaagacaaacatgtggcgtaagatggcactttgactaaaactacatacaagtggagatggcactaacagaaagtgaccatttctacatgggatgagatatatcaaggaattcattgacagactcagtcttacagaatctctatacatcaaaggtatttgccaactatccctcttctgaaaggtcaagaagtcaaaatccccatgaaaccttgaatggcggtacattaaaaaacaagaaccttcaaaatatgtaatagctcttttcagagctgtcatacacaaataaatacaaaatctactcttacttgctttccttcaatagtatcacaaaaggaggtactatgttgattcagtatatagtttgtatactcacaatgcatggaaaaatgcatggagaaccatgcatacagaacgttttacctcacgtattctcaattgattttctaacttttgtttttagcaaccatccttcatcaaaaagatccaagtgttaaataaacaagtctagaattcacagtttgtactctccttgtgcttcctcgttttctgttatttcttttcggcttgggtaagcaaactctgttactgccacattcttttttttttccactgagaatagtttcccatgttttcaaaagagcacagttgtgtgatatgtgttgtggggggaagaggtgaaagaaagaggggggaagagaatatacttgtgtaaatatgaatagtgtacataaacatatatgaagacatggtcttctagacacagaagaaaaaagatacataaatgaacacaaagtgtggaaacacatgtgtagtcagatggatcagtgtccttagggggcaaggtttcaaagctcagtctacaaaaccattctaattaaaataacattttaatatccaattctgctttactttgtaagcattttctcccttctgtttgttttctttactaaagtcacagcaagggctgtgctgagcctccagttcatctaagctactcggtgcatgcccagacagcaagaaaatggtttctctggcaacaggaattatgtgaaatctctgtgtgttctcccccaccttccatctgattcctattcacttaagctcttcacatataggcaacaacgaggcattggaaatctaatgagcaattcaaatttattgagctagttcatggaggcgggtactgtgagcatcttcatttcctgtgtaccagggagcagagtgtgtttgttgtacgttatctgtattattcaagaaccatgcactgtcagcaaatagcccaaaccagataaaatcagatgaatatctaaaataagaagcatatgaggaatttacttccatcatggtaggagggaaatgcaaaggctttcaggtgccaaacacagctttgaattttccaaagatgctgagcgatggaagtcacaatgatttaaaacagcctcatattgtgtctgaaacccaagagggaatggcaagagctttgattaaattgctttgaatgtcagcttttttatttctaaggaatcatactgttcctccatgactaaagcgctagagttttcaatttaggccttataaacattccctaataatagttcatgatgagacctcttatatatgtttttctctgtagcctttgttaaggagagagtcctgtgtttagcattggcactaaggctgatatttactaagagagtttaatcaaatgggaattgatttgcttggaggaatcaggactaaggcaaattagctttattctttagagattgggagaatgtgggagggaaggatctatttttcttcggttccagtaaggatgaaataacagcaagaaatatactcagtaacataaagtagaaaatagagtgaattggaatggactcctgaaccggtttcagaatcattgtcctggaagtttaagaagaatatttgcttcttactgtctagaatattttagtaaactctacctgcaaggaggtatatttttaaagtttccttggttttatcattgtatatcttacctgttaaaaattaaggactttgtcaccaaaaagcaataggaaatgcctctttgcataaatctttaatctcaatctacatgatatagatttaagtaataactcaatgaaagcccaatttaaataaactttaacttccagtgaaagctgtaagaaagcaatgagcagaatgattagcctaatgacacaaatatagtaaatgattaactaaaaagcatagaagggtgaagataccaaagacagatgacagtaaaataatagtagcattataacaatgacttcattcatttcatggttaatctttagataataagaacatattgttttagataataagatagtttaaaaattctcaaataactggcatttttcctgggatataaaagtgccaataagtacagccaaaatttggaaaataaatacaaaatataagtcctacacagaagagacacctactgaagccataacactcggaattttcaatccagtcacagagcttttaggaaaagaacatcttggaatcataatttcattccagttagaaaatggagattcaacactcatacctaaaaccaaattgcccttcacgtggtaagtcagataagctgagactaggggctttgtgtatgtagctagtgcttgcttctgggaacagagaaattgttcctgtgtttctaaatgtggtaccccactgcaagtagtgtgtagtagaacgcataaagatttactgaagttttcaaggaatttctaagctctggtctgcagttcttttcccacagagccacctttcaattgtgacttttgctatgttttattttaattttatttaattttaccctttcttccaggaaaagttgagatggcttactattatagtgtatgcatgtatcaatccttgaaaacagtatttcttttaaagagaaaattgcctagaatcaggaaaatatcttgataaggcacttatggtagaaagcagaagatgagaacatgtgttagtaggagagaaagcaatgaaaaatagcaaaactgttcctaagttagaaattaatggcaattagtgggtggtggggaatacaaaaaagaagaaaggaaaggcagagtggcctttagagggaaaacattaaaaattttagacatctaatattcaattttatgttgttgctgtttttacaaaatctttctcataattcagaaaagtgtggtacattcacattgctgagcacgctgatttttatggaaatgtgtttatcatgtgtgcttaagaaagatcaatttccccatttggctatataccagagcagggacacagagtaaaaaacaaaaaagttgtagagaaaagtggttcaagacagaggtgtttatgaggatgtaagacccactggaagttcagagaaaactgaagaactatattgggcttttcatggggcacggaatccaatcttatttacagcttaaaaggtaagaggacctcaggtaactgttagcccaagccacagcattttgcagactcccaccttttataaactccggtcagagtggaaaattccaccagagactgaaccgtgaagaaacatcttgtgggacaggtcccaggcctaacccctaacccagtgaattccttccttatcagcagcccagcataccattcccaccccatttcacagcaacctcagacctctcccgcctggacctacaactgccccagcctgcaagcgggaaaggaggctcctgcgctcgctggtgctccccctccgcaggtctttgtccaataaacctgtgttaccgtcgagccgccctccttgtctttttttctccatcttaacagtaacatggaagttataccacacaacacagcacacacacacacacagagtgaaaaggtaaaacgttacaatttttaaaatcagaaacaggaaaggtatataattaagcaggatgcaacatctgggagaagaaaaatgccatatatcaatgaactgtgtacacttgggcaatgtaacattagtgggccagcttcaggaccttactatggtgaaaatctgctacaaatttccactctctttgaagtcacatggatgtgaatcgtgtgtgctttcaacgtactagctgtgaatgaacttaggctagagggtgaaaatatcggagccccaatattctcctttcctgtaaaatacagatagtagtatctactttaaacataaataataatggcaaatttttatttactgcaaactatatgtcaagctccaaacttacagctattatttatttagtttactccttgcaactattctttgaagtattattattttcattgtacaaatcaggaacctaagcctaatagaaattaaataactttcctaagcacagagcttgtaggtagtggagccattagagtggttcactagtactgacaatagcagtactagtataagtattagtactagcataagtactaatataagcaaatactgtgaaagtcagtttcaacttgaaattttcaattactgacttcgttttctacaatgggcaaacccaagataactctgtaatgatggatcctttgtaaactttacttcttgtcattctgcatttttttcactatttctttatttaacaagggtggaacgccttgctcatttatcatcatagctgaattcttattagagcaccagctaattcatgcttattaagtagaaaagcaatggcaactaggcttgatgcctaagtaggattcaagcctgtatctaaagtgacaaaaaacttataacgctgtttcagatcaactatagagtggcaggaataaataccattgtatatgctcactgtaaagctagattatgtttccagtgtagtcacaccaagtaggagcacataccgtccatctcagcactttgtcctctagaccaggggtcctcaacccctgggccatggactggtaccatcctattaagaactgggccacacggcagaggtgagtggcaggtgagtgagcaaagcgtcatctgtatttatagctactccccattccttggattaccgcctgaactctgcctgtcagatcagtggcagcattagactctcatagaagcaggaaccctatcttgaacagtgaatgtgaggggtgtaggttgtccgctccttatgagaatctaatgcctgatgatgtgtcactgtcccccatcacccccagatgggaccatctagttgcaggaaaacaagctcagggctccccttgattctatggtgcattgtgtaattatttcattatatattacagtgtaataataatagaaataaagtacccaataaatgtagtgtgcttgaatcatcccgaaactatccatccccgcacccccaacccctgtccgtggaaaaattgtcttccatgaaaccagtccctggtgcccaaaaggttagggaccactgctctagatgattcactggggacatacggttgccagtgacactgtagggtcttaccaggtctggtaaacccaacctttgttatgtcactgtgcttttatacttttcacttacatcaccatttggaaaagtgtagactaacaatacaatgagggtttgtgtgtatgtattgaataacagacttggcattagaaatgttgcatccttatgtctgtggggaaaataggatgaatatctagatttacctgaagaatttctctgcctccagctttccaacattctggagagccagtttccctataccttctatgtgaaccaattaataggatgttaaagaaaaaggtaagaatttgtttgaactcaaggatctgacacatgctgttccaatcaattttacattctaataaaataaacaattgaagtcttacaaatactgcatgtccaaataaaataatacccattttttgtataataaactaaagcttatcaaatagcttcccttaaggttgaaggaaaaaaaataaagaaaaaaaatccaactgtaagtgaccttcaaataacctaagcattgtgttggcaagtttagtaagactatgttctccaaaagtttacagaagtgacattgtcatcagtatgtctactgaaaaaggagtgagtgatagaaaccactacgtttaaaaaaatcatttagttagaattatgatcgtgtattggggtttatgcaggatcttgcacgaagaaaataagcaagttgcaaccctctttcttttactttcaacgacaaaggtcatgccaagggtttggaatcctattgctgctattaagagctctttctatgcattaaacttgtctcaccaaagcaggtgtttgacatatgaggggcctggctgcagtactatcaatagtttcattacaggggacttactctccaaacatacctttcctgtggacagaatttaatttgaaccatcttttctagagggtagttgtttgtgattattttcttgaaataagtaaaaagtttaaatagaggtgatatgcaactccagtttaatgtgtgcactaatctttcactttatataatttatcatctataattttagttattataaatatttagttaaatctactcggttatctttcattaactatgaactcataatctacaaaaatatatcaaatggctgcatttccacattttccagaatcatatatcatagtactgtggctagataagattacctaaaatgcagataaattcttttgtaaatatgtcaaaatatatctaattaactatatataaaattacaaataaatcctgccttcctaagagggataaatttagaagcaacatttggagaaacacagtactgacatctgataagtatgactttgtttttcccctaagctataaatagtaatagctaacactgaatgcttcctatgtgccagtcatacaacactgagtgtgtactaactcacttaatccttataatacacctatgagattcaaactattagggatctcatcttatggatgaagaaactgaggtacagaataattaacttgctcctagacacagctagtaagtgaagctgacatttaaatctggacagtatgggtctaaaatcagtcatcttaaccattagttgtataatttatttagatatataatttataatttataaaatattattcattacatgtcagaataatctcttacatttaataatgaagaccacgagaaatggtccatttgtggtacaggacaccaccatatacaaagcagcttactaatgtacagctgtcgtgggaaaagatgtttctaaatcatttgtaccctggggacactacatgccattttattcaaagtccatggagattaatttctcaaaggataagttgagaaaaaatcatcttttccttcatcagaaaaccaaataatcaacttttatttctcaaaggtaagaaagatcaaatagacaacccttggatctaacctgtggttccacaaaggatataaaaatagcaagtgtgatgaatggatcataaaattgttccttctggggaaattctgtgatttaatgccacacagtatgtaaggagaatcgcaacataattgattgaaatctgaaatggagatacagggggcctaatcatttttctagaagaactctgaagaaagagttggacctaacgtttaaaaagctaacatctaacattaactctagtaagcaattataccagtgcttaaaccaatattacataaccaagaaaaaaataggaaatctatgtattctgtttacatttttactcacccacactgtaccagttcttcctcatggctgggtcctctctaataaatggaatttttgtataacatcttttaggtcacctaagcagtgatgtataaaatcactgtatatgtatgtatatgcccagaatgtatatgcccagaaaaataatgaagtctctcagcatatagttagctatcacagagtgactaaggtagcataagaattaatctcaaataatcctactatttgtaggttcctttaaaaaaatcaatatgcctgtaccttcaagttaccaagggcatatgtatgacatatgtgggttacctgatactttagaaagcagagaatagatatccccttatcacagaggcaggtcccgggtagatgcagaattttgaaaggaacatattgaaatcttctaatttgtgcttatcttgaaattaaattcagtcttctagtcattccaattttttccaacctattaaattgtgagaaatctgcaaagaatttattgagaaggttctcaaagaactaagatggtagctttttactaagaaactgattatatcaaggctgaagggtaagatttgttcagacaagctttcctagctagcatccaatgagtattagaatttccaagtctaatttataaacccaaacataaacagataaaaataataatttttattttcttcaagagaagagaaaaatgtaaggtagagtgaagtaacatttagactcagaaaatttaaatcaaagaactgacataaacaactagcaaacttgattgtttagattttaataaaatgtattgtataatctattattacttttagtgagagcaaaatattatagaaaaacttttttatttgtaaaatatatcttgttccaaggaaataagtatacgtaattaactaacacccataaaaggtatgactctttaatgttgtcaatgaagatttaacataatattctataacaaatatagctcattctgctcttaaaacacataattcattacctcatttgaatgtattgtttaatctaggaaattgtataataaatagcagtaataatatgggaataagcaatgtagttttactttcaaaactaatatccaccagtaaaactaaaatttgaactgtgagaaggcgatatatctaatcatgacactctcaggaggaaatagcacaacaattttaacccattatttgtcatatttctgcatgggaacatgtttcaaaataggtttcataggcctaacacataacccaggaataatcgcacaagtaattttgagggtatattcatagtcacctttccatattcaaatgttacaaaatgaatttctaccaaagacactattttcattcttattagagttatttgctcaagactatagccaaagaaatatagatcttaaatctcatcatcaaaaaagcccagaactctggcttcattttcaggcacaataccacaatggcaaaacatcagtctcagtgtgatatatcagttaataacgtaagcagtaagacacgggctaaatttaacacatactcaaaacaacctctgttaaataatttaacatgaatgatattaaggacaattaaatacatttgtttcttagacagtttgtctaagagtcttgaactcttttgtgagaatccctgggggaacttaaatgtgggtacttatgttttataggattgaccaggaatagtctaaaatcagaagtcatagccctcctaaagccatatagcttaattatagaataatataatcatagaattatagttggcttatctagttgatgcgattcatattaaaggaaaaggaagatgtaagaatgtggaaattattgccaaagagcactcagtaaagttgctaagagaaaatggttagtaaatcccaggccaccttaagatattaagttgtctgttaagcattgcagtgatcaaggaagcatccatacttagaaacgcatgattaatcttttaaataatatcctaatattgtttaaatatactttgatttttcttcaaaacaaaagaaaaatgtaaactgttattttctttggtcaatatatatgtttataagatggccttataaattctattgctcattggatgctggctaataaaatacattcatccattttctttcaatcaaccatatttatttagcacttactaaattcaagaaggcctgggccctaacacatttgtaagtgtgggcagaggcctaggaatttgcatatttaataagaaccataagtgattctgaaacaagtaagcttctgaccaaatattgcaaaacattgataagggactgcttcaagggggagaggcaatgacaacatcatgaaggatgcagtatttgaggtatttctagaaaaataggtaaaattagggtatgtagagatagtatgaagggcaattaagaagaggaaagagactaagttaggcacaagagcaagagggtgtagagtgaggaaataaccagtggcctagattggctaacaataagaaaattagagagtaacagaagagatgactataggtcagagggaaattgatttggatcaggaatgtcaaaaccagggagtactgactctattaaatacatgacagggagtttctaaaatttcttgagcaggtaaaagcttaattcaaagtatagggagatagatgttgtgaaaggtagttgaagccatgggaggaggtaaggttgctggggaggcaaaacagaacatgacgaagccacactcgggaataacattgaggagtgtctacatttgattgcctggagaaagaggaaaaaagaaggaaaactgggtgataatgttaccaaaatagcaggggtgtggtctaggtcctgctgcttgctgcacagaaagtcaatcactgagacaatgagtactgccagggaagaaggctttaattgggtgctgtagctgaggagatgagagatcacaatgaaatgattaaaaggataactaaaggaaatgtatagaagaatgaaaaggttgagtcaggggcacagcatagtaacatgtaggaagagaggatatagacattacattgcctggggacatctctttccctctctaggccactagcataggttcaaaacagagactaaattgcaatgcttatattctgtgtagactaaagactgaaaaagtaatggagctttactaaaagatgggtttcaaatgagagagtcagatgaaagtgcaagggatttccagcacctatgatggtaccatagttgtagatggcaggaaagcaaggagcagaagctttcaagtcgagtgcacagtcattttaaaaatgagaaggtgcaggaaattgatgagggagtttacagaacccaactgtctcacaatttgcattaaagtatgggcgcccttatttagtttgtggagttctctattctggcccttagttctattgctcctgttgaggaggaaggagaagaaaggttgcctgctcctgtgtgcctctttgaggtgccaggagattactctgaaatgctttcctagcatgtagcatgtcttgtacagcaattccagcactgagacatgtaccctgagatatgccaacacacttccagctggtccaaggctagaccacctaacttttgagtttcaacttctaataacaatgcataacagcacttgccagttgcaccattttacttcagaaggatgtcacatgaatcattgaaggagtgactttagaagaccttgagccaattggagagaagcgctctaagtgcccaataatttctcatttttaatattcagtgaagatttttgaaatgttaaagaaaaaaatagaggaactaggaataacaaatggctagcaggacacatttactggaatgaaggaggattgcaaagctattttctcaattatattttttacattaaaacaacgttgcatttttaagccctgcagataaaatgtcttttatgaagaaaagctaattaagtttcctgaaaaataaggcagctggttaacaatttacgtcttttttgaagcgttaacgcttatggtttttagggcccaagttactaagttaatctataagtgaatccaaaggtgaactaatagatcgaaaaatggttcatgcttaggtgtggatttctgagcactaaaaaaatttaaaaaatgaccatagaactattttgatcttcacttttgaacaaatcaggtttatatgttgtttcctttctaaaccttccattgtactttttaaaaataaatccccatcacagcactgaaaacacgcactatgcaactgtttaccaagtattaactgtgggtcaggcactatgctgaatgacagaaatgaaaagttaaactaggccaggcacggtggctcacgcctataatcccaacactttg

SEQ ID NO: 18953 - RNA, 1487 nt, Homo sapiens
  source 1..1487: mol_type = other RNA
tgcggggacaggccagggcatccctgaatgtcaagtatttgtttcacccgctgtcctgtaggactgtcggcaatagtgaagccgaagccctgggcacctttcacaatggttaaggtcataagttcagcttgggtggccccagatgaagccatagacacattgtcatcatggacgggcggtggatacgtgccgtctagctgaccatcagttggcatggagtgcagagaatgaggcggccgatctgttatatctggaactgactgtgaggtccgagaaatgtactccaaatatgtttcatagttgtgtcttccattgaccatcactggaggtggcctctccattattgcaaggggtggcaccatgctgttagcagggtcttcaggatcaaagggcaaagggtagccacgacacaacaccaggttgacactctgaccaataggaacagactggaaaagtttgacaacatctgcatgagtgtgtccaaggacacaaacttcattaatatagacaatgacatcacctgtttccatttttccatcctgtgctgcaggcccatccggaatcacacttttcacctgcagaaactcatcaggctcgtctccaccaatgatggtaaatccaaagcccatgttgctcttttttagggtggtgctgaggaatgttcccttcaactgggatgcatcccgggtgaagagtggtttttcgaacagccagggcctccctgctgggtcgcgctgatagtaagacaagtcattcacgctgcgcgacctctccggggcagcacgggggcggatggatttgggcctaggtaatgtccatgaggagctgtctactcggaaacctggggcctgcaggggctttgttccaagttctgtgtggggcatgttatgttgctgtagcttcctttttgcttccaggacaggattttcaaactgtgttcttctatttatgtggtcaacataataagtgccataaatgggatcatcgattttttcccagccatatggaagctcattttctttgcactcttctggaggtttagcctttttcgcaagtcgtggatccagccatgatgttgtctttgtgttatggtggttctaagtagccctgaaggaggtgtaagagtaattgtgcaaggcagctgtaaatttggcaacctcagctccctgtcctcaaagcagctatttttattaaaatcaactagaatgttgccaagttaacctcattgaaaatgcagaactcatccagagcaaaaggaatttattacaaatacaggattctccagttggaagagcacagtccacaggctctgataatgtttcctgagttttgcaaaagaattattttcatcttaaacctacccttttcataaacagttgttttgttactctttagctacagagctggcagaggcagtacaaaagtgatgcagattatagcatgttcttgggattcctgcattttctcaataagtgattaatagcaat

SEQ ID NO: 18954 - RNA, 2293 nt, Homo sapiens
  source 1..2293: mol_type = other RNA
tgcggggacaggccagggcatccctgaatgtcaagtatttgtttcacccgctgtcctgtaggactgtcggcaatagtgaagccgaagccctgggcacctttcacaatggttaaggtcataagttcagcttgggtggccccagatgaagccatagacacattgtcatcatggacgggcggtggatacgtgccgtctagctgaccatcagttggcatggagtgcagagaatgaggcggccgatctgttatatctggaactgactgtgaggtccgagaaatgtactccaaatatgtttcatagttgtgtcttccattgaccatcactggaggtggcctctccattattgcaaggggtggcaccatgctgttagcagggtcttcaggatcaaagggcaaagggtagccacgacacaacaccaggttgacactctgaccaataggaacagactggaaaagtttgacaacatctgcatgagtgtgtccaaggacacaaacttcattaatatagacaatgacatcacctgtttccatttttccatcctgtgctgcaggcccatccggaatcacacttttcacctgcagaaactcatcaggctcgtctccaccaatgatggtaaatccaaagcccatgttgctcttttttagggtggtgctgaggaatgttcccttcaactgggatgcatcccgggtgaagagtggtttttcgaacagccagggcctccctgctgggtcgcgctgatagtaagacaagtcattcacgctgcgcgacctctccggggcagcacgggggcggatggatttgggcctaggtaatgtccatgaggagctgtctcggaaacctggggcctgcaggggctttgttccaagttctgtgtggggcatgttatgttgctgtagcttcctttttgcttccaggacaggattttcaaactgtgttcttctatttatgtggtcaacataataagtgccataaatgggatcatcgattttttcccagccatatggaagctcattttctttgcactcttctggaggtttagcctttttcgcaagtcgtggatccagccatgatgttgtctttgtgttatggtcaatgaagtagacttcgcccttctctgtataggccatttcccagttatcaggcaatgggtctggttcctcattgtcttcaggtttagttggctttgtgtcatccatctgctccttcagctcctcaggctgactgtacactggtgcaggataaggctgggagggcatctcccctgaggcacctgcacttttgtcttcatgttcactggattctggtgttactactactccatttccattgaccacaggcctctcttcctcttcctcctcaggaggctctatactggctttctccatgttgctcactgatttattcctcttccgttttccttcagcacttggagtggctcctggaagtatctggtctgttacatttaacaataatggtgctggttctgctggcggctttggggtaccgtagtaattgtcttcataagtcccactttctaggagagcaccacttttctccaattccataaaatcttcaacagtgatgaaaatataatccactccagggacctcaccctccttatgtggccttgtggtgcatggcaccgtgcggaggtagaggttgtcacgaatgatttgctgaagctcatggtccacagaacccttttgaaatcgtaagttgaggtagtgacgaaggtctttatcaacaattcctccttgcttgacacacttgagccggagggggtccttgcagtgtttgatcacggccagcacgtccctgatggtgagccccgccacgggggtctcgttcacctccagcagcagctcctccgacaccaatttgctgccgctctcataggccaccttgccgggcttcacctcccccaggtaggggaactgtccattctcggcgccccccttcagttcaaagcccagctggccctccgggttcctgccaatgacactctcatggactttgctagtccagtggcttttctttttcaagcttttggacatggcagtggggcgagtcgcctcagttcctgggctccttggggttaggggggctggtggtgagagaatgaggatggaggagcaagggggcccagggggaagaacagcagactttgccttcgcccccctctattcggtgctttccctcttctttggatggagtgtggacgaggaatggggaggatgagagggacggctgggcagaggtaggagagcttggatgaggttgtgctgtcccttga

SEQ ID NO: 18955 - RNA, 2167 nt, Homo sapiens
  source 1..2167: mol_type = other RNA
tgcggggacaggccagggcatccctgaatgtcaagtatttgtttcacccgctgtcctgtaggactgtcggcaatagtgaagccgaagccctgggcacctttcacaatggttaaggtcataagttcagcttgggtggccccagatgaagccatagacacattgtcatcatggacgggcggtggatacgtgccgtctagctgaccatcagttggcatggagtgcagagaatgaggcggccgatctgttatatctggaactgactgtgaggtccgagaaatgtactccaaatatgtttcatagttgtgtcttccattgaccatcactggaggtggcctctccattattgcaaggggtggcaccatgctgttagcagggtcttcaggatcaaagggcaaagggtagccacgacacaacaccaggttgacactctgaccaataggaacagactggaaaagtttgacaacatctgcatgagtgtgtccaaggacacaaacttcattaatatagacaatgacatcacctgtttccatttttccatcctgtgctgcaggcccatccggaatcacacttttcacctgcagaaactcatcaggctcgtctccaccaatgatggtaaatccaaagcccatgttgctcttttttagggtggtgctgaggaatgttcccttcaactgggatgcatcccgggtgaagagtggtttttctcggaaacctggggcctgcaggggctttgttccaagttctgtgtggggcatgttatgttgctgtagcttcctttttgcttccaggacaggattttcaaactgtgttcttctatttatgtggtcaacataataagtgccataaatgggatcatcgattttttcccagccatatggaagctcattttctttgcactcttctggaggtttagcctttttcgcaagtcgtggatccagccatgatgttgtctttgtgttatggtcaatgaagtagacttcgcccttctctgtataggccatttcccagttatcaggcaatgggtctggttcctcattgtcttcaggtttagttggctttgtgtcatccatctgctccttcagctcctcaggctgactgtacactggtgcaggataaggctgggagggcatctcccctgaggcacctgcacttttgtcttcatgttcactggattctggtgttactactactccatttccattgaccacaggcctctcttcctcttcctcctcaggaggctctatactggctttctccatgttgctcactgatttattcctcttccgttttccttcagcacttggagtggctcctggaagtatctggtctgttacatttaacaataatggtgctggttctgctggcggctttggggtaccgtagtaattgtcttcataagtcccactttctaggagagcaccacttttctccaattccataaaatcttcaacagtgatgaaaatataatccactccagggacctcaccctccttatgtggccttgtggtgcatggcaccgtgcggaggtagaggttgtcacgaatgatttgctgaagctcatggtccacagaacccttttgaaatcgtaagttgaggtagtgacgaaggtctttatcaacaattcctccttgcttgacacacttgagccggagggggtccttgcagtgtttgatcacggccagcacgtccctgatggtgagccccgccacgggggtctcgttcacctccagcagcagctcctccgacaccaatttgctgccgctctcataggccaccttgccgggcttcacctcccccaggtaggggaactgtccattctcggcgccccccttcagttcaaagcccagctggccctccgggttcctgccaatgacactctcatggactttgctagtccagtggcttttctttttcaagcttttggacatggcagtggggcgagtcgcctcagttcctgggctccttggggttaggggggctggtggtgagagaatgaggatggaggagcaagggggcccagggggaagaacagcagactttgccttcgcccccctctattcggtgctttccctcttctttggatggagtgtggacgaggaatggggaggatgagagggacggctgggcagaggtaggagagcttggatgaggttgtgctgtcccttga

SEQ ID NO: 18956 - RNA, 2275 nt, Homo sapiens
  source 1..2275: mol_type = other RNA
tgcggggacaggccagggcatccctgaatgtcaagtatttgtttcacccgctgtcctgtaggactgtcggcaatagtgaagccgaagccctgggcacctttcacaatggttaaggtcataagttcagcttgggtggccccagatgaagccatagacacattgtcatcatggacgggcggtggatacgtgccgtctagctgaccatcagttggcatggagtgcagagaatgaggcggccgatctgttatatctggaactgactgtgaggtccgagaaatgtactccaaatatgtttcatagttgtgtcttccattgaccatcactggaggtggcctctccattattgcaaggggtggcaccatgctgttagcagggtcttcaggatcaaagggcaaagggtagccacgacacaacaccaggttgacactctgaccaataggaacagactggaaaagtttgacaacatctgcatgagtgtgtccaaggacacaaacttcattaatatagacaatgacatcacctgtttccatttttccatcctgtgctgcaggcccatccggaatcacacttttcacctgcagaaactcatcaggctcgtctccaccaatgatggtaaatccaaagcccatgttgctcttttttagggtggtgctgaggaatgttcccttcaactgggatgcatcccgggtgaagagtggtttttctcggaaacctggggcctgcaggggctttgttccaagttctgtgtggggcatgttatgttgctgtagcttcctttttgcttccaggacaggattttcaaactgtgttcttctatttatgtggtcaacataataagtgccataaatgggatcatcgattttttcccagccatatggaagctcattttctttgcactcttctggaggtttagcctttttcgcaagtcgtggatccagccatgatgttgtctttgtgttatggtcaatgaagtagacttcgcccttctctgtataggccatttcccagttatcaggcaatgggtctggttcctcattgtcttcaggtttagttggctttgtgtcatccatctgctccttcagctcctcaggctgactgtacactggtgcaggataaggctgggagggcatctcccctgaggcacctgcacttttgtcttcatgttcactggattctggtgttactactactccatttccattgaccacaggcctctcttcctcttcctcctcaggaggctctatactggctttctccatgttgctcactgatttattcctcttccgttttccttcagcacttggagtggctcctggaagtatctggtctgttacatttaacaataatggtgctggttctgctggcggctttggggtaccgtagtaattgtcttcataagtcccactttctaggagagcaccacttttctccaattccataaaatcttcaacagtgatgaaaatataatccactccagggacctcaccctccttatgtggccttgtggtgcatggcaccgtgcggaggtagaggttgtcacgaatgatttgctgaagctcatggtccacagaacccttttgaaatcgtaagttgaggtagtgacgaaggtctttatcaacaattcctccttgcttgacacacttgagccggagggggtccttgcagtgtttgatcacggccagcacgtccctgatggtgagccccgccacgggggtctcgttcacctccagcagcagctcctccgacaccaatttgctgccgctctcataggccaccttgccgggcttcacctcccccaggtaggggaactgtccattctcggcgccccccttcagttcaaagcccagctggccctccgggttcctgccaatgacactctcatggactttgctagtccagtggcttttctttttcaagcttttggacatggcagtggggcgagtcgcctcagttcctgggctccttggggttaggggggctggtggtgagagaatgaggatggaggagcaagggggcccagggggaagaacagcagactttgccttcgcccccctctattcggtgctttccctcttctttggatggagtgtggacgaggaatggggaggatgagagggacggctgggcagaggtaggagagcttggatgaggttgtgctgtcccttgaatgacactcaaggctgtggccccgcagcagaggaagcagtggtggtggcgtcggcggcggcggcggcggcagccggagcgagcagtagccgagctggtgagcgggtgt

SEQ ID NO: 18957 - RNA, 5730 nt, Homo sapiens
  source 1..5730: mol_type = other RNA
tgcggggacaggccagggcatccctgaatgtcaagtatttgtttcacccgctgtcctgtaggactgtcggcaatagtgaagccgaagccctgggcacctttcacaatggttaaggtcataagttcagcttgggtggccccagatgaagccatagacacattgtcatcatggacgggcggtggatacgtgccgtctagctgaccatcagttggcatggagtgcagagaatgaggcggccgatctgttatatctggaactgactgtgaggtccgagaaatgtactccaaatatgtttcatagttgtgtcttccattgaccatcactggaggtggcctctccattattgcaaggggtggcaccatgctgttagcagggtcttcaggatcaaagggcaaagggtagccacgacacaacaccaggttgacactctgaccaataggaacagactggaaaagtttgacaacatctgcatgagtgtgtccaaggacacaaacttcattaatatagacaatgacatcacctgtttccatttttccatcctgtgctgcaggcccatccggaatcacacttttcacctgcagaaactcatcaggctcgtctccaccaatgatggtaaatccaaagcccatgttgctcttttttagggtggtgctgaggaatgttcccttcaactgggatgcatcccgggtgaagagtggtttttctcggaaacctggggcctgcaggggctttgttccaagttctgtgtggggcatgttatgttgctgtagcttcctttttgcttccaggacaggattttcaaactgtgttcttctatttatgtggtcaacataataagtgccataaatgggatcatcgattttttcccagccatatggaagctcattttctttgcactcttctggaggtttagcctttttcgcaagtcgtggatccagccatgatgttgtctttgtgttatggtcaatgaagtagacttcgcccttctctgtataggccatttcccagttatcaggcaatgggtctggttcctcattgtcttcaggtttagttggctttgtgtcatccatctgctccttcagctcctcaggctgactgtacactggtgcaggataaggctgggagggcatctcccctgaggcacctgcacttttgtcttcatgttcactggattctggtgttactactactccatttccattgaccacaggcctctcttcctcttcctcctcaggaggctctatactggctttctccatgttgctcactgatttattcctcttccgttttccttcagcacttggagtggctcctggaagtatctggtctgttacatttaacaataatggtgctggttctgctggcggctttggggtaccgtagtaattgtcttcataagtcccactttctaggagagcaccacttttctccaattccataaaatcttcaacagtgatgaaaatataatccactccagggacctcaccctccttatgtggccttgtggtgcctagagctctgttcaaaggaagcagagaagccgcacgtcctctcccacctttccatggtcctcagtcagtgtcttctcaaaccacctgtactgatccaacccattcgcagataaaaataattttcttgatagaagtagtctcagctgagctttgatttttcaacatggatgtctagaattttcctctttaagccagacacagcaacacaaaactgccgctgagctcttttgttttccctcctctcaaagatgaagcatgcagcacttctctctctctctctctgtctccctctgcctctccctctctccctctccctctctctccttctcccctctctcgcttatgctctctccctccgtttccctttccccaacccccaccagcaacctcgctcgcttcccggtcagtcaggggcatttacatctctcagcacaagaacctgtgttatctacgcgcctgtctctcacttttgggtttcctctgggaaagggaggggggcggctctaggtgaagtcaggtgacccctccattaaaagccagtgagatggatggagtgtgtgaattttaatatacacacaggcacatttacattacaaagcagcgaggaaaatctagctcctagagattaagcatttttgtttttgctttcatagtccccttttaccaattaagagaagctagtatagtataatgaaatgtaattaaacttttcagtgttaataacaaggctgtatcctttcagaatcatccagctgaacaattcttttaaacttgtaagcatgactgtttcttttcctttcaagggtcaaagaatcagtcattttactacttacacactttttcaaattggtcttttctttgacatccatttaaacttatcttgaagttaaggaccattgtaaaagacaataaaaataataatgtgaaaggaaaaaaaaataagtgacaaaaacaccaaagcacatagcataggtagaaatcaatagtttgctgttgtggaactagattcaataatgagtaatgctttgctctgagacaaataatttttcccttctctgtttcagtgtctctgtcttaaatagaaaataaatgtaataaatatagcaagtatcctcttcttgcaacccaatcaagcaagcctagtagagaagggtgtccagatgctaagaccacacagcaccccagagacagaaacaactggaaaaacttgtgctaacctagtatagtattgaagatacatttatagtctatggacctaggccctaaagagtaaatttgacaccatcttctcctctgctgcaaagtttttaatatccagtggagaccatctcttctatctctaccactgaatagaaaagatacgtaatctgctgttaggaatactgtaaagaaaaatgagataatatccactttctttcaagggtcaaagaatcagtcatttttttgaacactcagataaaaagtactttgtaaggctaggtgataaattattagaatgaagaccaacaagcatcagaagaaaactcttatttggcatttggtgttctgtccacggattcttaattcaggagcatgatgatactggtgcctcagcaaaagaggaaaatagaggaagagctgacatagaatcacattatccttgccacaaaagataacatttcaaactcttacacaaacagcctctccctccttccagaatgatgttggaagagtgttgcatttgctgctgggactgaggactgcagccgaaatacacccagtcccctccatcaacacctaaaatgaataagaactattcactgttcttgctggctttgtatttgcaaagctttaccttgcatggaaaagatcccatttaagcttttaaaataaattatatgctaactggctgcaaatttagcttcagtttgtgctacaaaaattggcaccaaaacattggacaataaaaaaatcttccctcgaaaagtaagtcggcttaggcaaatttagaaagacctaaaatgttataggaaaaaaacataaaagatttcactttatagcttctaataaccaaatctgctgttctttcaccttttcttttttccctctagcattggctgttttcattttgcatttattcagagttttgttttgtttgttttccctacttcacccactggcttttgttcttttggccatggagtcactttccttgaatgtgcaaaatgtaggcaaggacagacagtgagaaagacatattaccttagatcagataatttgtgagctttaaccctaacactagtgtattttctgagaagaccacaggcaggacagacacacctaagcatatccaatacagacacaactttcaggctccaagctattctaacagagacttgatgaacatggaatatggactgcatgtattttctattaaaaacagaaagatcatgacttaaagaagcctattaaaacttaccaaagacaggccagtcccaaaaaaaaaaagattgatataaattggcaaaaacagtatagcaactaaccctagccaacttttcaaaatgccttccattactcaaggaacaaactgaagtgctgacagagggtagaataaatgtttactaatgcactcatttattcaactaatgttcactgagcacttcttttgtgctaggcaccatactaagcactgaggggtacaagaaaaagaaaacagagtgtttttcagaaactcaaaacaggtacccattaacatgtaatagatgttggtacaaagtgctatggagtgtcagaaaaagaagaaaaattctccttaaggcgaggcaggacagtcacatagaataggtaaccctcgaactgagcctttaagtatgtgtcagttttctaggtaagtaaaggcagggggttttcaggcagagacacaaagaacacgaacaaacctaaagggctgcgagtgatcttaaatgttctgccaaggaatttgtgcttcatctgagatgtaatggcaagttatttaaagttctttggctagacaattacatgttttacaaagattattttagcagcaaggtgaagggcagatgacagcagtgttttccaaactttcctaattataagaattacctgcaagttatagtaaatatatatatcactgggttccactccaaatctagagaagtccaagaatatctatttttaagcagtatcccaggcaattattattatcataaaatttctggaaacactggttttgtagtgtttgctgagtaccagaatcacctgtagagattttaaccaatcaaatgcaggccacctctaaattacttgaatcagaacatctggggatagaaaccggaaacattgttgattttaatcttctaaggtggttccaatgcatccgaggttggtaatcattggtttggagagaggcaagacagaaaaaagactatttagaagctgttgtagaggatatttgggtgaaacaacagaattcaactagctcaagtaaaggagtactcgtgctacaaaaggcaatatcataaacataggaaacacagtaacgctgtacgaagcctcacaggaactggggctaagaagccactaaaaaccaagaatcctcttctctctctcagtggctgtataattcacttctttgattcttcctgtctcttatcctgaaccagctttcttttcttgcatgctgtcatctccagggccatgttgccttgtcagttctcatgtcagcaggcaaagactggattggttgggctgatttccttagtttgccactgatctcatcagttatagccagagtgtctcacattcactttgcaggagctctgggcaaagattttctgagaagaccacaggcaggatagacacacctaagcatatccaatacagacacaacagttcaagcaaaaaatgcttaagaagacttgagtaggctagtggtagaagagactaaaggtcccagatgcttttcagaggtggaactcacagaacatggtgactaattgaatatgagggtgtggaagagaaaaagtcaccgcagaagaataaatatattttcatttactgcagatgctacattataatacaaacaccactaagtgactatccattttactagtcagtagaggatatatatttggttttgaactccacacttacatatatatagaagcctaaaggtcagggccgggcgcagtggctcacacctgtaatcccagcactt

SEQ ID NO: 18958 - RNA, 1022 nt, Homo sapiens
  source 1..1022: mol_type = other RNA
tgcggggacaggccagggcatccctgaatgtcaagtatttgtttcacccgctgtcctgtaggactgtcggcaatagtgaagccgaagccctgggcacctttcacaatggttaaggtcataagttcagcttgggtggccccagatgaagccatagacacattgtcatcatggacgggcggtggatacgtgccgtctagctgaccatcagttggcatggagtgcagagaatgaggcggccgatctgttatatctggaactgactgtgaggtccgagaaatgtactccaaatatgtttcatagttgtgtcttccattgaccatcactggaggtggcctctccattattgcaaggggtggcaccatgctgttagcagggtcttcaggatcaaagggcaaagggtagccacgacacaacaccaggttgacactctgaccaataggaacagactggaaaagtttgacaacatctgcatgagtgtgtccaaggacacaaacttcattaatatagacaatgacatcacctgtttccatttttccatcctgtgctgcaggcccatccggaatcacacttttcacctgcagaaactcatcaggctcgtctccaccaatgatggtaaatccaaagcccatgttgctcttttttagggtggtgctgaggaatgttcccttcaactgggatgcatcccgggtgaagagtggtttttctcggaaacctggggcctgcaggggctttgttccaagttctgtgtggggcatgttatgttgctgtagcttcctttttgcttccaggacaggattttcaaactgtgttcttctatttatgtggtcaacataataagtgccataaatgggatcatcgattttttcccagccatatggaagctcattttctttgcactcttctggaggtttagcctttttcgcaagtcgtggatccagccatgatgttgtctttgtgttatggtggttctaagtagccctgaaggaggtgtaagagtaattgtgcaaggcagctgtaaattt

SEQ ID NO: 18959 - RNA, 461 nt, Homo sapiens
  source 1..461: mol_type = other RNA
tgctatgccaacatattgccatctgatgagtccgtccagaatcttcctgccacttaattctctaggatctcctaagtgtccacacagagccttgggcggtaggatcccaggaatggaaccggatctaggcggggttcctgacacaacacccatcttctggttctccctgtggtttcccaagttagtggagatggccctgatcccaagccaggcgcagcaccaatgcagatttcttgccacagaaaaactatgggagatggaaaggcgtcctgagaacagaggagctccagtgctgctgtgtttaaagacggcaggagcaaggccaagatagggagctgtgagtggccctgagccttaaccttgagtcctcatttattgtaacatcgaactccaggatccatcccagtggacacgggaaagggaggtatcgagatgcacttggttttctctgcagtgtgttc

SEQ ID NO: 18960 - RNA, 379 nt, Homo sapiens
  source 1..379: mol_type = other RNA
tgctgaggtccgggctgtgccctggctgggagcgcgacggaccagaagcgagcagacgcgcggctaaccccgggactggccccgcggcgctgtcacccagggccgctcttactttcctggtccgaaagtagctcgcccgcgagggagtgtgcgcaggggcggggcgggaggggagatgaccagaaagggtggcgtggggtctcctccccacagtccgccgatcctcctcctcctgcgggcctcgcttccttcttctccactggacgctccacccgccccttttccagtccctgtccccaaatgcagggggtaaagtactcaagaagagggggccgggaaatggaaaaacagccaggcacgggacgagtggcaagcagtt

SEQ ID NO: 18961 - RNA, 385 nt, Homo sapiens
  source 1..385: mol_type = other RNA
tgctgaggtccgggctgtgccctggctgggagcgcgacggaccagaagcgagcagacgcgcggctaaccccgggactggccccgcggcgctgtcacccagggccgctcttactttcctggtccgaaagtagctcgcccgcgagggagtgtgcgcaggggcggggcgggaggggagatgaccagaaagggtggcgtggggtctcctccccacagtccgccgatcctcctcctcctgcgggcctcgcttccttcttctccactggacgctccacccgccccttttccagtccctgtccccaaatgcagggggtaaagtactcaagaagagggggccgggaaatggaaaaacagccaggcacgggacgagtggcaagcagttgcgaaa

SEQ ID NO: 18962 - RNA, 672 nt, Homo sapiens
  source 1..672: mol_type = other RNA
tgctgaggtccgggctgtgccctggctgggagcgcgacggaccagaagcgagcagacgcgcggctaaccccgggactggccccgcggcgctgtcacccagggccgctcttactttcctggtccgaaagtagctcgcccgcgagggagtgtgcgcaggggcggggcgggaggggagatgaccagaaagggtggcgtggggtctcctccccacagtccgccgatcctcctcctcctgcgggcctcgcttccttcttctccactggacgctccacccgccccttttccagtccctgtccccaaatgcagggggtaaagtactcaagaagagggggccgggaaatggaaaaacagccaggcacgggacgagtggcaagcagttgcgaaacgatccgcactggagcaggaggagtagaagcagaggggagggagtccgagggggcggaggtggagtgcagcggggccgaggccgcggagcccagagcggacagcctgagcccagcggccgctgtcagcaggctcaggcgcggggcgcgccggggctccgacgagcgtgcgcgcccgaggccggcttccctccggcgggcggcagcggctccggcgaagcgaggcaccttggcggcctcgcgctgctcacgagcccgcgcggcttcaagacggcgcggcgagagaaag

SEQ ID NO: 18963 - RNA, 1111 nt, Homo sapiens
  source 1..1111: mol_type = other RNA
tgctgaggtccgggctgtgccctggctgggagcgcgacggaccagaagcgagcagacgcgcggctaaccccgggactggccccgcggcgctgtcacccagggccgctcttactttcctggtccgaaagtagctcgcccgcgagggagtgtgcgcaggggcggggcgggaggggagatgaccagaaagggtggcgtggggtctcctccccacagtccgccgatcctcctcctcctgcgggcctcgcttccttcttctccactggacgctccacccgccccttttccagtccctgtccccaaatgcagggggtaaagtactcaagaagagggggccgggaaatggaaaaacagccaggcacgggacgagtggcaagcagttgcgaaacgatccgcactggagcaggaggagtagaagcagaggggagggagtccgagggggcggaggtggagtgcagcggggccgaggccgcggagcccagagcggacagcctgagcccagcggccgctgtcagcaggctcaggcgcggggcgcgccggggctccgacgagcgtgcgcgcccgaggccggcttccctccggcgggcggcagcggctccggcgaagcgaggcaccttggcggcctcgcgctgctcacgagcccgcgcggcttcaagacggcgcggcgagagaaagagcgctcggctcaggcgaagcctcttctgccgtccccaggcctccgtctcctcctccggcgcctcctcccgccgctccctccgcctgccagcaccccctccctggcgaagccccctcctcgctggtcccacacctccctctagcgactccaagcctgtcccttcgtggatctctcgcactccctcctttggttgcacacacgagcacaccagtctagggagaaaccaggtgggtggaggaggatgtgcgggggagaagactggaggtttgggtgaatgaggcgagaagtcacagttacccatttaaacccgcacagagaaggctgcctcaatctggggctgactgagcgggaagatgcagggcaactcgaggatggcccggggcagccgccctgggtcgcggaagcccacgcccctgttttgggcgccgggcagcaggg

SEQ ID NO: 18964 - RNA, 66 nt, Homo sapiens
  source 1..66: mol_type = other RNA
tgctgaggtccgggctgtgccgggcgctgggggaagcgcccaccttccaggtgggaccgcgggaag

SEQ ID NO: 18965 - RNA, 48 nt, Homo sapiens
  source 1..48: mol_type = other RNA
tgctgaggtccgggctgtgccgggctctcgccccggcctgagggtcct

SEQ ID NO: 18966 - RNA, 403 nt, Homo sapiens
  source 1..403: mol_type = other RNA
tgctgaggtccgggctgtgccgggctctcgccccggcctgagggtcctcatggggctgggggctgcccgatgggggagctgggcatgagcctgagggtgtgggggaccctcctgcctctggagcgcgcccgatccctcccgtcttggaactcccggggcttttgtggagcgcggcgcggtggtggttctgggcgtttcctgcccgggggcggttggcggggcgcgaggaccaagttaagagtctgttgcaccccagccccggggcaaagccggggatccctggctccgcgtcccactggcagcgcggggagggctctggccgccgcccggctcttcgcaccgcagcgcagcgcggctcagctcccggctcgttgcggctgcttcggctccgcgcggggaatgc

SEQ ID NO: 18967 - RNA, 71 nt, Homo sapiens
  source 1..71: mol_type = other RNA
tgctgtattgtcaggtagtgataaatcctatcactacctgacaatacagcagtatgtgttttattttctat

SEQ ID NO: 18968 - RNA, 223 nt, Homo sapiens
  source 1..223: mol_type = other RNA
tgcttcctttctcagctgaacccctgctcccggagcctccaggagtgccctctgaggtggagctgcagcaccctttccgggagccagtggtcagacaccatttcacctgtgaccaacagatgcactctctgagaccccaagggaaggggctgcactccacctctctgccctgtttgttctgtgtatgcctctacaataatgctcacctcttgccctcaggttg

SEQ ID NO: 18969 - RNA, 69 nt, Homo sapiens
  source 1..69: mol_type = other RNA
tggaagactagtgattttgttgttgtcttactgcgctcaacaacaaatcccagtctacctaatggtgcc

SEQ ID NO: 18970 - RNA, 2386 nt, Homo sapiens
  source 1..2386: mol_type = other RNA
tggaagactagtgattttgttgttgtttgagacagggtctctgtcgcccaggctggagtgtagtggcaccatcctagctcactgcagcctcaacctcccggctcaagtgatcctcccgcctcagcctccctagtggctgggactacaggtgcacgccaccatgcctggctatttgttgttgttgttgttgttgttgttgttgttgttttgtagaattggggttttgccacgttacccgggctggtcttgaactcttaagctcgagtgatctgcatcttggcctcctgaagtgctgggaatacaggtgtgagccagtgagcccaacccacagtgatttttaagaactgtttctttgtggaaaatgactccttccaaaagttaaatgctccttcatggagctgaagagaaagtgaagagattaagggtagcaatacttcttagccacaaaacatgagtttccctgacttgatctttgacttggctctttactgatccagccaaagctgaagccagggcactgggggagcatgacagccttgccagagagggaggccggcccacccaggaatgcccatccaatcggtccagactgggatttggagcctgtctgtggcctactggctcagtcaccttgggcaagtcatttaacttctctgagccatcagcttttcatttgccaaatgaggatggtgatactatctgccttgcagggttgtcgtgagggttacatgggagagctgtgtgatggctaccatcatcacatcttcatcttcatcatcatcaagtgtttaggcctcacccgggagcaacggggccagtaaaaagctttctgcccggtgtgggaaggttggacttaggagttggacaggccactctagaggtcaatgtggagaggggactggccactccagttgaccttcctgagtagtacccttaggcatgaattggactgacccagcagaagtttggcccaggattgtggccgagaaacaaaatctgaatgtaactaacacagctttaccttatccacttgcctgggatggtacttatgctaatcctattccaagcaaaagcaactcaaactaataaaagctgcgcctccgctctgggttccacaccatctgtcggtccacacgcttgggattagctcttcccatggagcccagactgtctgctcggctgcgtggactatcagaggccagcctggaggcacgggggcggtgccatccattcatgagcacatatgcatggagccctgcatggggccaagccctatgccaaggactggaggtccagtgaaggagagacggacaaggtcgctgctcccaggaagagctctgcagggtggtgaaatatagtagtaacttcatctgactgacatgggggaagtttagaggtgtccttggcatattcacagtgaaatccatcaccctttcaccatgttgggtgatagcaaccgtatggcgcttcctagtgacagccagtgtgcgttctgttaggcagcaccagcgcactgcagctaatgaagcacattcctgcaggcctgtctcctagggctctccgaatcctctgtctgcaaaggaacggcaccatgggaaaatctagcacagccagcatcagccatcacccaaactcaaaagcgtctttgaacggcagagacaggcccattttcctctctgcctggcccagggctggaaccgtcctcaggtcactttttgtgggtctgtacaaacgtgccgactggcagcgagccgctcttcacctgagcccggatttcagctcggtgctttaatgtgaagaccagggctctcaccgtccgccggtacggcccattaatgaggcgggagcagagatgaaacgtttcccgttcaatattttcaaccagtaggtgatccatctttaattccaaggcttctgagagtaatttctgagcatttttcctcaacgactcggttttgggatcacttctaacttcaatagaaggtctatttgaatgtttttcagtgaaagttttccactcagtgtaaacttctctggcaagagaagccacttctgaatctgagtgtttacgcatcttgttcacagtgtgaccttcagagattcaatcgtggcctgcttgtaaacctttcctccagaatctttcttctgagggctattctggattctaggcgttcgaatgacgaatttatccattgttaggggactccgactaccttgacgtgcttgcagcgtgttcaggaaaagcagccctggtagctgctgttggcgccctccagactgcaacctcgtaggctcccaagcccagtcgtctgtgttgaaactaaacagacgcttcctcccagggcggtagttcctctgaagaaactccgccggccctcgcgcctct

SEQ ID NO: 18971 - RNA, 5549 nt, Homo sapiens
  source 1..5549: mol_type = other RNA
tggaagactagtgattttgttgtttgcaagacaacctaaaaaatatctctggaagatatcagatgtcttaagaaaagcttgtgatgatatttcatatcaaaacagtaagcaagtttcctgtggtcagctaccattccctttaataaattacttaattaattcattaatacttatttctattccttaaaactcctggacccaggcatactcaagtatgtcttaataaataccttttgactttattcctggaaagattacccatccttaatgtggccccctaagtgtcagaaaaagaaaagactccctttgaatgactttatttatacttctgcatttagcatactacagactatcaaaattttacatattctacagagttaaaagaagatgtatactgtggcttttaaaatattagccttatctgttgttacagagcaaaatagctctaggttcagtaattcactcctatcctcttttgaccagtggaggaagttgaatattctttggctttgtaatttcctgggaaatttgagtaattggggtaaattctttaaaagttgtatataattcacaactccagggcaaatttttttctaattttattttgtcatatagagtttcattttagtgagcttatagtaacattgtatttaagaaagaaaaaatttctgtaccatgcaatagtaaatttacctttttcttagaatgctttaattctttttagagatttttaattgggtaatactacatagcaaacacacagaaatgatatatcataaataggacattactaaattttgaaactagaaaaatatgttatactatataatttggacactacctataaatcagcatatataagccaagatcttattgacaaatcaaatcaggaatttaaaatttatgctagtgagaaaaattagagggtgagataaactagcagaataggtttctattattatttcatgcttatcaacaccatattgtcaattctgctaaaggttcctggttgattcctgcaaaatggcagcagaggtttgctaaagcaaccactactttacttactaaaagcgaataattagcatggtattactttacagaagaattcttttccaactttcaccattaaacattttacatgttctaaaaacatttttttagatccccttaaaaaaaaattccccaaagcttaagcatactacaagctgctgcttcttttttttttgtccacagctcggcctatgtaaatcattttaacttcagagctatgtaataaagagctggatacgaatgaatatcacctactaaaaacaaaacctgaaaacacaattcagttcccatctgcttacttggaaggtcatttgccactagtgatgacaaccatgtcaggcctcacttgcttcaattcgagaagtaaacttagtgagttttgctttcttaagtcaaaaccacagtggtaaagggaaagacgagtgtgatattcctcaacctcaccagtaagcaatattcgtcaagactacatctatcactaaacacacactagaatcagaagaatccttgactccacaggagatttaactgaggccccacattaaggttcaggctcaggcattgctagtttaccctgaagaaacctcatcctattgccactctctaatggaattttcctcctaggaaacacttcctaatttggaatttattttctctagtgcaataattaaggtaggagtgcttgatggcttgtggacttgactatgtagtcaaacttaaaaaaaatggttaacccttgtataaatctgtggttgaatttttatttatgttatctgtgaaaccaacagggcatctggcacacattttagatttttcccatagatatgaacatatattgcatatttagttctttttgaattttgctcgagctatatggaaaagcaaaacagagcaaggagaatgatgccaattgccatcgtaaggccagttacatgctggagatggactacaggccactcaggcacaaagaagactctgcctcaagttttagttccttagtcctaatataagagaaaagtttatgaatgctaaggagagctctcccctagcagtggtgtttccatttatttttctcattgtgatttctcaccttgctcctagatgacctgagcacgaagttgtgcgttataaatcacattgttggttttttagtggtgggaattggatctaaaccacaatgactatgaaaaagtgagctggggtcctgactacttgctatattgcacggtactatactttgtgattcgacttcgagctgtgctaggggaggcggacccaatggtttggttaaagtgatggtcagaggaactcctcatgtggccaatgctggctgtccctcccaagctgctcaggccaatgccaccaccacttatgccagctccactcagggcaccgctcccagcacccatgctggtgccaaccaggccactgctgcctatgccaccgctgatcccagtggtgccactaattccagttacgccagcaccagaaacaaccctctctgtcacaatgacattgtgggcattggctaactcggggtgcatactcagactacctatcatgccggaagttggttggattactctttctgtcactaccacatttgaagactctctaggatgatggatagtcagagaggtgggtagactagagcttggtgctattaccctttctgtcactataacattcgacccatctcgcaagtcaggcatctctaacattccatgcaaatcagcgccagagattgggccgaccactctctctgtcactaccacgtttgatgctggtcggttatcgtgaacgtgcacagagggcttcagagtgtcagaggtggtgtaagactcggtcacagtgacattaccatagcccagaggatcgagaataggcttaggatgcagtacaccaggtcccgagggataggtgctctcagaaattactgtggtagtgccgaaatgtggggagattggtgggtgtccactaacaacgggctctgtttcctgaggaaggcaaactggttcagtgctttgtggtggccaagaaggatcaaggtctggatatgattcttttcctaggctgatgtctgccaacttcttaaatttaggtcccagggtatccaagaagctgtcatccaggtcttctccaatgaagctacaacaacccacagagccagcaggggaacctacaccttcgatgtcatatatgagcaaacagtcattagatgggcgtccttcatcttcatctgcgtaagcatatgctttctgacagaagtagctttccatgaaattcatattcagacctccttctctacattccctcatagaatttcttcttaatgttccagagtattcttgacatatctcaggcattcctgaagttttaactccctctgttagttcaaatcctgtcattctctctcctcctcccagatcttgcatttctctgccaccatactcatttgtataaactcctgagttgtcaatgcattcaattatatttgcgttatcaggtggtatttgtggtatgacagtggttatatccctgggttcaggctgtggtccttctactgcccatgaatgaattgctccatctgaacattcgggaacaggctcaaagccagctgcactacgaggagcacctccacaatcacaacagatcatcaaaaatgggaccaatcctaagaccaagaatcccatgatgaggagtccaatgccagcaggaccaaaatgtacattgtctgataacaaatctttggctccgtttccgggttcagaagaatatacttggctagagtcagtagaagttgtgctggtatcatagttagtggaagaagtactttcttgtctgccagtattggtagtaattttagtgttcggctctgtattagtcctgtcgtcattaccaaaactttgaatgttaatattaattgtaccagtgcaagttctttgaagattatcatctatagagagaatcgttccttggtattttcctccgagcatattgtactgttccttggtaactttatttttcaaagtgagtttgcctgttcttgaatcaacagctagcaggtcagctggattatttcccattacatacctaacagtcgttgaaggtctacctgtgtccaggtcagtagctacaaagtctcccactttatcatttgatcccatattaccagttacaacatatgtctttgaacctggacgaaacactgggccttcaattacatttaacacagtcacagaaattgcagatgctttcagtttatattgagacataattgaatgatgaaattcagctttatttctgacaccaatactgagttgcagactctgcatagcttcataatctaagggcttaacaacctttaaaattcccacatttgttctttcattcatttctatctcaaaccaatttccttcatttccagagataaagaaaattactgccatccagttagctgagaactcttcatccaaatcaattactctaatctcgagcaaatttgaatttagagtattttcttgaatttctatggtatatgaagactgttccatgtaagggatattatcattgacatcgaggattttaatgttgcactcacattccgctgacatgccatctgccccgccatctcggtcagagcctcttacagcaagagcatactggccgtattgctctctgtctagaaaattattcatcgttcgaatttctccagtatttctgttgataataaacattggtgaatctgaaggttcttgtcttataatcttgaaggctatttttgagttcaaattgttcggttcatctgcgtcagtagcattgagtatcatcaccagtgtatttgcattagaattttcttctatttgtcctgcaaatgtagccattgaaaacactggagggttgtcatttatatccaaaaccctgactctgagctctagaggcctctctaaatcttggcccattgagttcagagctcggcagtagataatgaagaaaggagtgacctctcgatcaactatggatgttatattaatttcaccagttttctgattaatgacaaagatcccatatggtggctgatcaattcctactccagagatgcggtatgtaacttgctggtttgcagcacaatctgagtgaattttggcgattgggttcctctttgagttgtcttcaccttcacgacaggctgctgcgaacttgatccattcacgtttctgccttcggattgaatgccatttgatggtgccatttttagtgttataatctcttacctggattcggaattcactgttaacttctaccaccaccagaaaaatgaacagcattgcaactactctgaagaaactccagtccatctctgctggattctcttacatccaagaccaagggagttttgtttgttcttctctgttctttttctttctcccactcagctggtgtctgattaaaataatttctcagtagatgttcttacatgcaggctttgaggtgtttct

SEQ ID NO: 18972 - RNA, 72 nt, Homo sapiens
  source 1..72: mol_type = other RNA
tggaagggagaagagctttaatgattggagtcattttcagagcattaaagctcttctcccttccatattaat

SEQ ID NO: 18973 - RNA, 73 nt, Homo sapiens
  source 1..73: mol_type = other RNA
tggaagggagaagagctttaatgctctgaaaatgactccaatcattaaagctcttctcccttccatattaata

SEQ ID NO: 18974 - RNA, 4760 nt, Homo sapiens
  source 1..4760: mol_type = other RNA
tggaatgtaaagaagtatgtataacaattatgttttgttgaagatttgcaggagcattgtgacccaaccaatgacaaagaagttcccaacctccttggactcttgctggcgcccagatgtctgtggtcataggtcacctcttcatcccaactctgtcctcttccctttgcccttaacataaaaagagccgagcccaacatttgtactgacttaagatggtactttaggacagtagtctaccatcgtctcagtttgctggctctccgaataaatctgcttttcctcgcaccaattttcttctctcccgagttttggctttggagccgcaagcagctgaaccttggtttggttacaagtttgcattctcattatgtgagaaatgggaggcagggtaaacttaggtagagcacaggcctcacatacttagagctacagagctcccagactcactctgggttccttgtttcctggaggaaaaaaactaggtttccaatcccagttgcctcagtgcctcatgtgtgcaactccaatgctggggttatgaaaaaagcctaactaagcagtcctcaacttatgagtaagttgtttttcaactgttcatttgcctttctctcttgtgaactcaagaaggtttttccacacagaaagtcatgtaagttccaatcccagaagccaatttgacacctaatatacctgaattataatacttataccattatgacttctatgggaatatgtgttcatatttacaacttagctagaaacataatattcctataggaccagagacgcttctagttccaacccagggatgaaattctatacagggtttatggctagagaggcaagagacaggggcactaagaaaatggggctggggagtatattacaggagtgaagagaagatgggacaaagacacagggctgtgtagaaaggtaattaggagtgggacttactaaggaagaatgcagattacccttcttttatttttccccttccccttttgtcactgtctcaccacttcaaacccactaaccagctagaagtgtgaagagaagagaggactggagttgtgttggggtgtagtaggaagttagtcccagaaactgtggagtttgctgtggcagggtagaaaaggaaggaaataacaggccatctcagtagagattaagaatgatttctgtaaataaaaagacagatcaggagccatgtgtacttccatgtggcttatctgttgtccactaaaataatcaagacaggttctcatccaaagcagaatttttactcagcaaggcaaggttagagtcaaccagttttggttgattcatttttcagaagcccaagggatagtatctctaatttggggtccttttatgtgctcaagaagtaaacaaaccaacaaaatgtaaatcagttctcaagagccattattagggaattcagaacatagtgctaacatgagatctgagaaataaaagaaggtaaagcataaaacagagaagagcaccaggccctcccctaaataaacaaacaacacaaggccttgcactcagaagacccttggaatgtaggtctgtctctctttctttgaatacttaaatctgaagggatggaaagaccacctaaaaatcctagttttttggcatgatgggggtctaattccttgttcactccaaagagctgatggcacatgttccctgtaaggatctccttgtgctaaaagtctgcagtggcctttagtttataggactgtgttcaggcttccccacttcgcagacagccatgaagtcagctgtcattcaactcaacgcttctcaaattttaaagtatattaagtaactgtggagctataaaaatgaagattctcaactcccatcctaggcctaatgaagcagaatgtgagtgggattcagggatgttaaacaagctccaaacatgattttgatgttcatcaaagttggaggatcactagagtaatggccaggactagaagtcaaaagacctgcacttaggttactggtctttttctttgtgtgggattatagctatgttgccatctccataggcaagagtattctcatttttaaaatggagaatgcttttgatttaccaaggtattttaggaattgagaaaagtgctctgtaaatgtccaagtgctataaagtattagatgaaattattcacactctggccctcttatgtgtctgtccccaagctgtttccaacttaatgctattgattgcccaatttgcacgaaccttttacttcaggttggctagtcttttccctgatgcttccaaaccacatgcactcttatgatggcttacatttgttttacccgctttctcccttttgactgctaagtctgcccgtcaaatccttattttaaataaaatctttcttgaccactccaggcaaaagtaacctgtcctttagaatttacagcacttatagtctgttacaaagtaccactttcattcgacaccatctggtgcatcaattctactctcctgtagtcttatatgactaaatatgtggatcttatctatcccaaactaggctacaaactctctgagaaaagagtttggggttatcttcttgttctccacagcacgtagtacaatgggcagcacacagtgaattcttattaaatatctgaggtttccttataacaatggtgactgaagttttgccccaataattgtaaagctaaatagtatttctcaccggcctgaactctgtgagataacttccctgtagtcatcacacagaaacagatttttctcctttgtggatagtctgatgttgagtaagagctgagttctgcctgaatgatttcccacactctttacatacataggtaccacgtctattatggattctctggtgtttactaagatctgacctctgtctgaaggcttttccacactcatcacattggtagggcttctccccagtgtggattctctgatgctgaatgaggctggtgattcctcggaaggcattcccacactcatcacacttgtagggcctctctccagtgtggattctctgatgttccgtgaggactgatctttgagtaaacgccttcccacacttatcacatttatagggtctttctccagtgtgaattcgctgatgttctgtaagacttgtcctttgaataaaggctttttcacatacgtcacatttgtagggtttttccccagtgtgaattctctgatgctgaataaggccactctgactgaaggatttcccacattccttacactgatagcatttttctttgtggtggatttcctgatgggaaacaagggatgagttataaacaaaggcttttccacactcgttgcactcatacggcttggcgccggtatgaactccttgatgctgagtaagtatggaacgccgactaaaacttttattacactgagtgcactgataaggtttgtctcttgtgtggatcttgatatggtgaaagaggcctgctttctgactaaaggctttgccacagtcattacagtgatagtgtttttctcctgtgtgaagtctctgatgttggttaagagctgaccaccggccaaaggctttgccacattcattacacttatacggtttctctccagtgtgtattattttgtgtcgaataagcacagttctcccacggaaagcttttccacattcttcgcatttgtagggtctatctccagtatggatcctctgatgttctatgaggtgtgagtgctgactaaaagcttttccacagtcatcacatccgtaagattcttctcctggacagattctctgatgttcagtatggtcagagttctcagtcaggcttactccattttcatcacaggtaggttgtttatcttctctggagcaagcagagggctcttctgttatttcttcaggttcacgagtttctccacacctagcagacttggacatatcattttcaaatttactggatgtcttcccatgtggttccatttcttcagaaacttcttgctttaaattcccatactcatttccagtctcaacatctaaaacttgctcctgttgggattcaagttctggagattcatactttggctgggctttcatggactggagggacatactgggttctccttcttttcgtagacgtaccgtctcctgcaagaacatttcctgttccccagtgtggactgagacctgctctcctggttcatccagttctctctctaaatcctccagcacagtcaccacctcctccccactctctggatgctgctcctgcacccaggcctggagctcctcaggtaggatggtcaggaactgctccagcaccagcagctccagaatctgttctttggtgtgggtctctggcctcagccactgatggcaaagttctcggagtcggctcaaagcctcacggggaccagatgtctcctggtagcagaactgtctgaagtactgacggaagacctctctgctatgggtgttgtttttacgcaggtcccaatcctgtctggtggtatatttctcttcctctatctttacttccaaaggttcatcctggtccatgtgggcctggatagcccaagtagatgccattttagctgtgctagaactaccggtgtttcaagtaagatctcacctggaaactgtattcctggacagtcctgcggcccccagggccagaagagaactccctcctacggagcgaaggcaagaggcctcgaacccttttgggacccggaacccatcaaaagt

SEQ ID NO: 18975 - RNA, 4781 nt, Homo sapiens
  source 1..4781: mol_type = other RNA
tggaatgtaaagaagtatgtataacaattatgttttgttgaagatttgcaggagcattgtgacccaaccaatgacaaagaagttcccaacctccttggactcttgctggcgcccagatgtctgtggtcataggtcacctcttcatcccaactctgtcctcttccctttgcccttaacataaaaagagccgagcccaacatttgtactgacttaagatggtactttaggacagtagtctaccatcgtctcagtttgctggctctccgaataaatctgcttttcctcgcaccaattttcttctctcccgagttttggctttggagccgcaagcagctgaaccttggtttggttacaagtttgcattctcattatgtgagaaatgggaggcagggtaaacttaggtagagcacaggcctcacatacttagagctacagagctcccagactcactctgggttccttgtttcctggaggaaaaaaactaggtttccaatcccagttgcctcagtgcctcatgtgtgcaactccaatgctggggttatgaaaaaagcctaactaagcagtcctcaacttatgagtaagttgtttttcaactgttcatttgcctttctctcttgtgaactcaagaaggtttttccacacagaaagtcatgtaagttccaatcccagaagccaatttgacacctaatatacctgaattataatacttataccattatgacttctatgggaatatgtgttcatatttacaacttagctagaaacataatattcctataggaccagagacgcttctagttccaacccagggatgaaattctatacagggtttatggctagagaggcaagagacaggggcactaagaaaatggggctggggagtatattacaggagtgaagagaagatgggacaaagacacagggctgtgtagaaaggtaattaggagtgggacttactaaggaagaatgcagattacccttcttttatttttccccttccccttttgtcactgtctcaccacttcaaacccactaaccagctagaagtgtgaagagaagagaggactggagttgtgttggggtgtagtaggaagttagtcccagaaactgtggagtttgctgtggcagggtagaaaaggaaggaaataacaggccatctcagtagagattaagaatgatttctgtaaataaaaagacagatcaggagccatgtgtacttccatgtggcttatctgttgtccactaaaataatcaagacaggttctcatccaaagcagaatttttactcagcaaggcaaggttagagtcaaccagttttggttgattcatttttcagaagcccaagggatagtatctctaatttggggtccttttatgtgctcaagaagtaaacaaaccaacaaaatgtaaatcagttctcaagagccattattagggaattcagaacatagtgctaacatgagatctgagaaataaaagaaggtaaagcataaaacagagaagagcaccaggccctcccctaaataaacaaacaacacaaggccttgcactcagaagacccttggaatgtaggtctgtctctctttctttgaatacttaaatctgaagggatggaaagaccacctaaaaatcctagttttttggcatgatgggggtctaattccttgttcactccaaagagctgatggcacatgttccctgtaaggatctccttgtgctaaaagtctgcagtggcctttagtttataggactgtgttcaggcttccccacttcgcagacagccatgaagtcagctgtcattcaactcaacgcttctcaaattttaaagtatattaagtaactgtggagctataaaaatgaagattctcaactcccatcctaggcctaatgaagcagaatgtgagtgggattcagggatgttaaacaagctccaaacatgattttgatgttcatcaaagttggaggatcactagagtaatggccaggactagaagtcaaaagacctgcacttaggttactggtctttttctttgtgtgggattatagctatgttgccatctccataggcaagagtattctcatttttaaaatggagaatgcttttgatttaccaaggtattttaggaattgagaaaagtgctctgtaaatgtccaagtgctataaagtattagatgaaattattcacactctggccctcttatgtgtctgtccccaagctgtttccaacttaatgctattgattgcccaatttgcacgaaccttttacttcaggttggctagtcttttccctgatgcttccaaaccacatgcactcttatgatggcttacatttgttttacccgctttctcccttttgactgctaagtctgcccgtcaaatccttattttaaataaaatctttcttgaccactccaggcaaaagtaacctgtcctttagaatttacagcacttatagtctgttacaaagtaccactttcattcgacaccatctggtgcatcaattctactctcctgtagtcttatatgactaaatatgtggatcttatctatcccaaactaggctacaaactctctgagaaaagagtttggggttatcttcttgttctccacagcacgtagtacaatgggcagcacacagtgaattcttattaaatatctgaggtttccttataacaatggtgactgaagttttgccccaataattgtaaagctaaatagtatttctcaccggcctgaactctgtgagataacttccctgtagtcatcacacagaaacagatttttctcctttgtggatagtctgatgttgagtaagagctgagttctgcctgaatgatttcccacactctttacatacataggtaccacgtctattatggattctctggtgtttactaagatctgacctctgtctgaaggcttttccacactcatcacattggtagggcttctccccagtgtggattctctgatgctgaatgaggctggtgattcctcggaaggcattcccacactcatcacacttgtagggcctctctccagtgtggattctctgatgttccgtgaggactgatctttgagtaaacgccttcccacacttatcacatttatagggtctttctccagtgtgaattcgctgatgttctgtaagacttgtcctttgaataaaggctttttcacatacgtcacatttgtagggtttttccccagtgtgaattctctgatgctgaataaggccactctgactgaaggatttcccacattccttacactgatagcatttttctttgtggtggatttcctgatgggaaacaagggatgagttataaacaaaggcttttccacactcgttgcactcatacggcttggcgccggtatgaactccttgatgctgagtaagtatggaacgccgactaaaacttttattacactgagtgcactgataaggtttgtctcttgtgtggatcttgatatggtgaaagaggcctgctttctgactaaaggctttgccacagtcattacagtgatagtgtttttctcctgtgtgaagtctctgatgttggttaagagctgaccaccggccaaaggctttgccacattcattacacttatacggtttctctccagtgtgtattattttgtgtcgaataagcacagttctcccacggaaagcttttccacattcttcgcatttgtagggtctatctccagtatggatcctctgatgttctatgaggtgtgagtgctgactaaaagcttttccacagtcatcacatccgtaagattcttctcctggacagattctctgatgttcagtatggtcagagttctcagtcaggcttactccattttcatcacaggtaggttgtttatcttctctggagcaagcagagggctcttctgttatttcttcaggttcacgagtttctccacacctagcagacttggacatatcattttcaaatttactggatgtcttcccatgtggttccatttcttcagaaacttcttgctttaaattcccatactcatttccagtctcaacatctaaaacttgctcctgttgggattcaagttctggagattcatactttggctgggctttcatggactggagggacatactgggttctccttcttttcgtagacgtaccgtctcctgcaagaacatttcctgttccccagtgtggactgagacctgctctcctggttcatccagttctctctctaaatcctccagcacagtcaccacctcctccccactctctggatgctgctcctgcacccaggcctggagctcctcaggtaggatggtcaggaactgctccagcaccagcagctccagaatctgttctttggtgtgggtctctggcctcagccactgatggcaaagttctcggagtcggctcaaagcctcacggggaccagatgtctcctggtagcagaactgtctgaagtactgacggaagacctctctgctatgggtgttgtttttacgcaggtcccaatcctgtctggtggtatatttctcttcctctatctttacttccaaaggttcatcctggtccatgtgggcctggatagcccaagtagatgccattttagctgtgctagaactaccggtgtttcaagtaagatctcacctggaaactgtattcctggacagtcctgcggcccccagggccagaagagaactccctcctacggagcgaaggcaagaggcctcgaacccttttgggacccggaacccatcaaaagtgacccacaaaggccggaagcg

SEQ ID NO: 18976 - RNA, 4846 nt, Homo sapiens
  source 1..4846: mol_type = other RNA
tggaatgtaaagaagtatgtataacaattatgttttgttgaagatttgcaggagcattgtgacccaaccaatgacaaagaagttcccaacctccttggactcttgctggcgcccagatgtctgtggtcataggtcacctcttcatcccaactctgtcctcttccctttgcccttaacataaaaagagccgagcccaacatttgtactgacttaagatggtactttaggacagtagtctaccatcgtctcagtttgctggctctccgaataaatctgcttttcctcgcaccaattttcttctctcccgagttttggctttggagccgcaagcagctgaaccttggtttggttacaagtttgcattctcattatgtgagaaatgggaggcagggtaaacttaggtagagcacaggcctcacatacttagagctacagagctcccagactcactctgggttccttgtttcctggaggaaaaaaactaggtttccaatcccagttgcctcagtgcctcatgtgtgcaactccaatgctggggttatgaaaaaagcctaactaagcagtcctcaacttatgagtaagttgtttttcaactgttcatttgcctttctctcttgtgaactcaagaaggtttttccacacagaaagtcatgtaagttccaatcccagaagccaatttgacacctaatatacctgaattataatacttataccattatgacttctatgggaatatgtgttcatatttacaacttagctagaaacataatattcctataggaccagagacgcttctagttccaacccagggatgaaattctatacagggtttatggctagagaggcaagagacaggggcactaagaaaatggggctggggagtatattacaggagtgaagagaagatgggacaaagacacagggctgtgtagaaaggtaattaggagtgggacttactaaggaagaatgcagattacccttcttttatttttccccttccccttttgtcactgtctcaccacttcaaacccactaaccagctagaagtgtgaagagaagagaggactggagttgtgttggggtgtagtaggaagttagtcccagaaactgtggagtttgctgtggcagggtagaaaaggaaggaaataacaggccatctcagtagagattaagaatgatttctgtaaataaaaagacagatcaggagccatgtgtacttccatgtggcttatctgttgtccactaaaataatcaagacaggttctcatccaaagcagaatttttactcagcaaggcaaggttagagtcaaccagttttggttgattcatttttcagaagcccaagggatagtatctctaatttggggtccttttatgtgctcaagaagtaaacaaaccaacaaaatgtaaatcagttctcaagagccattattagggaattcagaacatagtgctaacatgagatctgagaaataaaagaaggtaaagcataaaacagagaagagcaccaggccctcccctaaataaacaaacaacacaaggccttgcactcagaagacccttggaatgtaggtctgtctctctttctttgaatacttaaatctgaagggatggaaagaccacctaaaaatcctagttttttggcatgatgggggtctaattccttgttcactccaaagagctgatggcacatgttccctgtaaggatctccttgtgctaaaagtctgcagtggcctttagtttataggactgtgttcaggcttccccacttcgcagacagccatgaagtcagctgtcattcaactcaacgcttctcaaattttaaagtatattaagtaactgtggagctataaaaatgaagattctcaactcccatcctaggcctaatgaagcagaatgtgagtgggattcagggatgttaaacaagctccaaacatgattttgatgttcatcaaagttggaggatcactagagtaatggccaggactagaagtcaaaagacctgcacttaggttactggtctttttctttgtgtgggattatagctatgttgccatctccataggcaagagtattctcatttttaaaatggagaatgcttttgatttaccaaggtattttaggaattgagaaaagtgctctgtaaatgtccaagtgctataaagtattagatgaaattattcacactctggccctcttatgtgtctgtccccaagctgtttccaacttaatgctattgattgcccaatttgcacgaaccttttacttcaggttggctagtcttttccctgatgcttccaaaccacatgcactcttatgatggcttacatttgttttacccgctttctcccttttgactgctaagtctgcccgtcaaatccttattttaaataaaatctttcttgaccactccaggcaaaagtaacctgtcctttagaatttacagcacttatagtctgttacaaagtaccactttcattcgacaccatctggtgcatcaattctactctcctgtagtcttatatgactaaatatgtggatcttatctatcccaaactaggctacaaactctctgagaaaagagtttggggttatcttcttgttctccacagcacgtagtacaatgggcagcacacagtgaattcttattaaatatctgaggtttccttataacaatggtgactgaagttttgccccaataattgtaaagctaaatagtatttctcaccggcctgaactctgtgagataacttccctgtagtcatcacacagaaacagatttttctcctttgtggatagtctgatgttgagtaagagctgagttctgcctgaatgatttcccacactctttacatacataggtaccacgtctattatggattctctggtgtttactaagatctgacctctgtctgaaggcttttccacactcatcacattggtagggcttctccccagtgtggattctctgatgctgaatgaggctggtgattcctcggaaggcattcccacactcatcacacttgtagggcctctctccagtgtggattctctgatgttccgtgaggactgatctttgagtaaacgccttcccacacttatcacatttatagggtctttctccagtgtgaattcgctgatgttctgtaagacttgtcctttgaataaaggctttttcacatacgtcacatttgtagggtttttccccagtgtgaattctctgatgctgaataaggccactctgactgaaggatttcccacattccttacactgatagcatttttctttgtggtggatttcctgatgggaaacaagggatgagttataaacaaaggcttttccacactcgttgcactcatacggcttggcgccggtatgaactccttgatgctgagtaagtatggaacgccgactaaaacttttattacactgagtgcactgataaggtttgtctcttgtgtggatcttgatatggtgaaagaggcctgctttctgactaaaggctttgccacagtcattacagtgatagtgtttttctcctgtgtgaagtctctgatgttggttaagagctgaccaccggccaaaggctttgccacattcattacacttatacggtttctctccagtgtgtattattttgtgtcgaataagcacagttctcccacggaaagcttttccacattcttcgcatttgtagggtctatctccagtatggatcctctgatgttctatgaggtgtgagtgctgactaaaagcttttccacagtcatcacatccgtaagattcttctcctggacagattctctgatgttcagtatggtcagagttctcagtcaggcttactccattttcatcacaggtaggttgtttatcttctctggagcaagcagagggctcttctgttatttcttcaggttcacgagtttctccacacctagcagacttggacatatcattttcaaatttactggatgtcttcccatgtggttccatttcttcagaaacttcttgctttaaattcccatactcatttccagtctcaacatctaaaacttgctcctgttgggattcaagttctggagattcatactttggctgggctttcatggactggagggacatactgggttctccttcttttcgtagacgtaccgtctcctgcaagaacatttcctgttccccagtgtggactgagacctgctctcctggttcatccagttctctctctaaatcctccagcacagtcaccacctcctccccactctctggatgctgctcctgcacccaggcctggagctcctcaggtaggatggtcaggaactgctccagcaccagcagctccagaatctgttctttggtgtgggtctctggcctcagccactgatggcaaagttctcggagtcggctcaaagcctcacggggaccagatgtctcctggtagcagaactgtctgaagtactgacggaagacctctctgctatgggtgttgtttttacgcaggtcccaatcctgtctggtggtatatttctcttcctctatctttacttccaaaggttcatcctggtccatgtgggcctggatagcccaagtagatgccattttagctgtgctagaactaccggtgtttcaagtaagatctcacctggaaactgtattcctggacagtctcagaaaaatactctgatagaaaagacttaagattagaccgatttaggccgggcacagtggctcacgcctgtaatcccagcactttgggaggccgagtcgggcggatcacgaggtcaggagatcgagaccatcctggctaacatggtgaaaccccgtctctactaaaaatacaaaaa

SEQ ID NO: 18977 - RNA, 357 nt, Homo sapiens
  source 1..357: mol_type = other RNA
tggaatgtaaggaagtgtgtggggtccctggatgacaccagcacccagtgcggctctgtctggcaaccgctcccaaggtggcaggagtgggtgtcccctgtgtgtcagtgggcagctcctgctgagcccgcagctcactggggagcctgacagcggggccatgtgcctgacactcctctctgcttgtggacctggcaaggcagggagcagaaaacagagccacttgaaggctttctgtctgcgtctgtgtgcagtgtggatttagttgtgcttttttcttgctgggagagcacagccaccatttacaagcagtgtcaccctcgtgggtggcgaggacagaacaggagcctctgctct

SEQ ID NO: 18978 - RNA, 1356 nt, Homo sapiens
  source 1..1356: mol_type = other RNA
tggacctctcctccccagtgtaacctcaaatcgtgggtcgttgaggcacagcacagaggagaatagggaggttctatcaggtggcctgccccagggtaagatagcagggtccagttgttcttcccatgtctcttcagctgtcctatggcttgttcagcgtgtgctttgctgttgatagtcttatcaccttctcctacaatgaagaggaattgcccctgggcctcttcaataggaaacaaatattgactggccccaacttgagttgtctcaaaagtgcgatagagctctagtaaccccaaggcattggtggatattaattgtgcagaatggggaaggggctgatggatctgaccatgatatacctgtggaatgccaaaaggaaagttggtcccattaataagtaccgtggctgtgacttgctttaggtaaatagccatagatagtccaatctgtactccttgacatacagagactaccccaacgcctgagccaaagacctttggatgtctcaggagaaagttggcagcctcctcaaaatattccaaatctgttacttctggtttgcggggcaggtcttcatagttatggtaagccaaggccaaggaggcgaagccacgactggctaggaggctggcccgaaattcaagcagcccacccaaaccaccaaacaaatcaattacccctgggaagagaccctctcctggagggagaaagagagctcctcgaaggcggccttctcgaaccttaattcgtgtgacaccaggtgccacataccacctctccaaagtcaggctggcctttggagcactggcaactttattgttcactattaactctaagtcataaagttttacttggacctggaaaggcctattcatcacatctcttttcaacagtcttgttaatagcttttcaggtttcagagaccagaagagacccatggggtggactcccatataatcccctccaagtgaagaagcatgattcaggtccacctcaccgaattcattggccctatagtgggcttgagaataaaacatgtctccgttttcatcttccagtgatgcctgaaaactcaccatctgaaagggaatcaggcctgtagctcggatatgcactggctcatcaacaagtgcactcacaggggtagctgtcaactggatcatttttttagtgtggcacctgggatgattcttcaggaatatcttcagcaaaacctcaaaacattattttaataattttctttatagaagttgtttgacccctattggcaccattagggcatatttttcttctgcaataaaatactcaaggtaacttctggagggctctgcatttgcaaatggtttctttcct

SEQ ID NO: 18979 - RNA, 1377 nt, Homo sapiens
  source 1..1377: mol_type = other RNA
tggacctctcctccccagtgtaacctcaaatcgtgggtcgttgaggcacagcacagaggagaatagggaggttctatcaggtggcctgccccagggtaagatagcagggtccagttgttcttcccatgtctcttcagctgtcctatggcttgttcagcgtgtgctttgctgttgatagtcttatcaccttctcctacaatgaagaggaattgcccctgggcctcttcaataggaaacaaatattgactggccccaacttgagttgtctcaaaagtgcgatagagctctagtaaccccaaggcattggtggatattaattgtgcagaatggggaaggggctgatggatctgaccatgatatacctgtggaatgccaaaaggaaagttggtcccattaataagtaccgtggctgtgacttgctttaggtaaatagccatagatagtccaatctgtactccttgacatacagagactaccccaacgcctgagccaaagacctttggatgtctcaggagaaagttggcagcctcctcaaaatattccaaatctgttacttctggtttgcggggcaggtcttcatagttatggtaagccaaggccaaggaggcgaagccacgactggctaggaggctggcccgaaattcaagcagcccacccaaaccaccaaacaaatcaattacccctgggaagagaccctctcctggagggagaaagagagctcctcgaaggcggccttctcgaaccttaattcgtgtgacaccaggtgccacataccacctctccaaagtcaggctggcctttggagcactggcaactttattgttcactattaactctaagtcataaagttttacttggacctggaaaggcctattcatcacatctcttttcaacagtcttgttaatagcttttcaggtttcagagaccagaagagacccatggggtggactcccatataatcccctccaagtgaagaagcatgattcaggtccacctcaccgaattcattggccctatagtgggcttgagaataaaacatgtctccgttttcatcttccagtgatgcctgaaaactcaccatctgaaagggaatcaggcctgtagctcggatatgcactggctcatcaacaagtgcactcacaggggtagctgtcaactggatcatttttttagtgtggcacctgggatgattcttcaggaatatcttcagcaaaacctcaaaacctagcaagagaacctgcccccaaaatttcagcgtaggttctattttccctaagtgtcggctggtctgagaaataaagagaaagagtacaaagagaggaatttacagctgggcctccgggggtgatgtcacatatcagcaggaccgtgaggcc

SEQ ID NO: 18980 - RNA, 1320 nt, Homo sapiens
  source 1..1320: mol_type = other RNA
tggacctctcctccccagtgtaacctcaaatcgtgggtcgttgaggcacagcacagaggagaatagggaggttctatcaggtggcctgccccagggtaagatagcagggtccagttgttcttcccatgtctcttcagctgtcctatggcttgttcagcgtgtgctttgctgttgatagtcttatcaccttctcctacaatgaagaggaattgcccctgggcctcttcaataggaaacaaatattgactggccccaacttgagttgtctcaaaagtgcgatagagctctagtaaccccaaggcattggtggatattaattgtgcagaatggggaaggggctgatggatctgaccatgatatacctgtggaatgccaaaaggaaagttggtcccattaataagtaccgtggctgtgacttgctttaggtaaatagccatagatagtccaatctgtactccttgacatacagagactaccccaacgcctgagccaaagacctttggatgtctcaggagaaagttggcagcctcctcaaaatattccaaatctgttacttctggtttgcggggcaggtcttcatagttatggtaagccaaggccaaggaggcgaagccacgactggctaggaggctggcccgaaattcaagcagcccacccaaaccaccaaacaaatcaattacccctgggaagagaccctctcctggagggagaaagagagctcctcgaaggcggccttctcgaaccttaattcgtgtgacaccaggtgccacataccacctctccaaagtcaggctggcctttggagcactggcaactttattgttcactattaactctaagtcataaagttttacttggacctggaaaggcctattcatcacatctcttttcaacagtcttgttaatagcttttcaggtttcagagaccagaagagacccatggggtggactcccatataatcccctccaagtgaagaagcatgattcaggtccacctcaccgaattcattggccctatagtgggcttgagaataaaacatgtctccgttttcatcttccagtgatgcctgaaaactcaccatctgaaagggaatcaggcctgtagctcggatatgcactggctcatcaacaagtgcactcacaggggtagctgtcaactggatcatttttttagtgtggcacctgggatgattcttcaggaatatcttcagcaaaacctcaaaacctggattcttcctcttgagccttcttttccagcagtagagggaaaatgacagacaccctaccaaaacttgcccagaaggccaaaacctcaaatat

SEQ ID NO: 18981 - RNA, 420 nt, Homo sapiens
  source 1..420: mol_type = other RNA
tggagagaaaggcagttcctgaaactgtcttcatcctcaatgtaagactccaggccactaacaaattcttctattattttgggataggaagggtgtctcctcagggtctgaaagagcttcttttggaaagctatttgatccacagctagttgattctgactctctcccgttttaagaataattcctgatatcttaagaagctttacaaagatgctgtcattttcttcaacttcattagcaatatgagatttctttgtctttttggaaagtggttgcttcctggttttggaggcatcttctgtcaggctctctttatcctcagattttgacagtcttcttttggaaaccattttgaccaatgtcttgtgcacttaaattacttccgagaagccgtcgccgcccgtagttttcgactttccc

SEQ ID NO: 18982 - RNA, 573 nt, Homo sapiens
  source 1..573: mol_type = other RNA
tggagagaaaggcagttcctgaaactgtcttcatcctcaatgtaagactccaggccactaacaaattcttctattattttgggataggaagggtgtctcctcagggtctgaaagagcttcttttggaaagctatttgatccacagctagttgattctgactctctcccgttttaagaataattcctgatatcttaagaagctttacaaagatgctgtcattttcttcaacttcattagcaatatgagatttctttgtctttttggaaagtggttgcttcctggttttggaggcatcttctgtcaggctctctttatcctcagattttgacagtcttcttttggaaaccattttgaccaatgtcttgtgcacttaaattacttcctgtggggattatcccatctcagggcagatgaggaagccaaggttcggggcgcggagccccagaggagaacgccgaccgcggcccggacttagagattaggccgcaggggagcggggcctcgagagactacgaccattgctccacttactcaccgagaagccgtcgccgcccgtagttttcgactttccc

SEQ ID NO: 18983 - RNA, 1489 nt, Homo sapiens
  source 1..1489: mol_type = other RNA
tggagagaaaggcagttcctgatgtgagtggcaattgctgagccacacaaagactgcagcatctgcggacgcactcttccaggagccagaggagcccacagcagcgtgggtctgagcgtgctgaggtggtgagcgtggatataagactagatcaggaaatggagggccaggcgaggtggctcacgcctgtaatcccagcactttgggagtccgaggtgggcggatcacttgaggtcaggagttgaagaccagcctggccaacatggcaaaaccctgtctctacctgagatgtagtttgtttctgtaaatttcagaagttgagttcagaatagacatatccagatttataagaatcacaggcttcttgctctcttggtgccacctcctggaacacgggggtggcatactgtagctcctgggagtgtttggcctcatcttgggctgtggaaacacacggcctggatcccacttctggcacagattcctcctttgcttgtttttcaaggatatttgcatagattccaacttccatggctgtgtctccacggtccctgggcacattatttctcatagcttttcttgttttgtatttgggcagtacccaaaaagccagaattaggattatcaccaccagcaacagtaataaccctggaagtagtagcttcagacagaaaggacagctgtctccgcctgttgagggcatggtgacagggtgactgtatgttgcatagttaggcaatctgtttttagcttcacacctatactcttcctcttctccaggattcttcttggttaagttaaattcagcaggctccctgtcatacttggaaatagctggtgatatggcaacatggttttcaaagaaagtgtaattgatgggcagcgagccattgactgagaggcaatgtaatgttatatgtcggtctgtttctgtttgaatgaccataatgttcagcactggggaagtcaccgggtcgacaatcgtgaagctgaagtcacgactgtattttgaacagctggtaacttgggctttgcatttgtaggggcctgattcatgggcttctgtgatgcttaggttaaaaatcgcaggttcaccttttccatcctgggttcccaggtgtgtcttacgtcgaaacaatgaataggtgatctgcagtgatttgttcttatgggaacaaaacatagatacattttgacccttcataaccaccttagtctttgagtccaaacatggagaagggaattcatttgttttcattgcctcacaatccaatacagcttttctacaagtgacagaagaaaatatgctccagaagaggagcctgttcaaatggctccacattctcccagttgaagtccaagacggggtcagaaggcatagtagaaccacagtggtgagtaactcggagaacttcctctttttcttagccaagttaaggaaatcagagggtttggatgaggtttgcataatactggtttgttcgaccaa

SEQ ID NO: 18984 - RNA, 1315 nt, Homo sapiens
  source 1..1315: mol_type = other RNA
tggaggagaaggaaggtgatgccttggaacagactttaacaactgtgaggcaggataaaaaacaagtcctgaaagccatcactttttgaccatagtgagctcttcttttgtaacggttcaggcttctaaccttatttcctcctttggcaactgaccagctcacgcacacatactagtgatgaaatccacataactccatatcttttcctctacatggccaagagtttcagtgcaacaggaaagtgctgtcacggatccatcgtgcaacacatacagtgctgtaaagcaaaggcctcgtctgcctgcaggcagcaggaactgcacgcattacccttctgtctgatgtacagcctaactgcttcgtgcttcttctcatgtgttgagccacagctttcttgtagagtatttcaaaaatacagccccaaaacaaagcataatcgaaagtcatcccaggtgaaagtggttggcttgggggaggtcacacagtcctttcagttcaggtagaatccttgtttctaggtcatttgaccaacatcatcccaggctccttagggaaatcaggagggggcagaagcaggctgaccagctacaggctacacacagaagaacgaaccttcccaaatttctggaaaaaatcttcttgtgcccgggccaaggcctcttcgtcaatgtagacagccggcctcttggccatgaggaaatactgcaccttcctcagattccagcccatcacatactggagccagccgcagacagccgcggtggagcggcccaccccagcgttgcagtgcacgtacacgatgtgtcccttctccagcagcgcatgcagcaggcacaccgcctggggcagcatctgtactcggccttcggtgctcatatctggtgttggcatccagatgtaggccaagccttcttccctatatagtttaatcatagtgtctggagtcatgggctctgggtagcggttacagcctgaggaattctgtacaatatcccattcagtctggaaattcattacagctgtaatccccaattcatgcttcagtttgatggttacatgttccacctgacgagggcagctacccagccagatatttggtagaattcttgaataatgcatggcttggtggcctgcaatattaaaatagaagtctgttgtgtgcttcatttcattggtgtgcccagtggcctcaatccagtgtcctattgggagacaatacacaccatccaccaagttgttttcattgtaagtacagcaacggtcatgatgaggtccattgcagagattaactagcttgcccaaggtcacaaaact

SEQ ID NO: 18985 - RNA, 1557 nt, Homo sapiens
  source 1..1557: mol_type = other RNA
tggaggagaaggaaggtgatgccttggaacagactttaacaactgtgaggcaggataaaaaacaagtcctgaaagccatcactttttgaccatagtgagctcttcttttgtaacggttcaggcttctaaccttatttcctcctttggcaactgaccagctcacgcacacatactagtgatgaaatccacataactccatatcttttcctctacatggccaagagtttcagtgcaacaggaaagtgctgtcacggatccatcgtgcaacacatacagtgctgtaaagcaaaggcctcgtctgcctgcaggcagcaggaactgcacgcattacccttctgtctgatgtacagcctaactgcttcgtgcttcttctcatgtgttgagccacagctttcttgtagagtatttcaaaaatacagccccaaaacaaagcataatcgaaagtcatcccaggtgaaagtggttggcttgggggaggtcacacagtcctttcagttcaggtagaatccttgtttctaggtcatttgaccaacatcatcccaggctccttagggaaatcaggagggggcagaagcaggctgaccagctacaggctacacacagaagaacgaaccttcccaaatttctggaaaaaatcttcttgtgcccgggccaaggcctcttcgtcaatgtagacagccggcctcttggccatgaggaaatactgcaccttcctcagattccagcccatcacatactggagccagccgcagacagccgcggtggagcggcccaccccagcgttgcagtgcacgtacacgatgtgtcccttctccagcagcgcatgcagcaggcacaccgcctggggcagcatctgtactcggccttcggtgctcatatctggtgttggcatccagatgtaggccaagccttcttccctatatagtttaatcatagtgtctggagtcatgggctctgggtagcggttacagcctgaggaattctgtacaatatcccattcagtctggaaattcattacagctgtaatccccaattcatgcttcagtttgatggttacatgttccacctgacgagggcagctacccagccagatatttggtagaattcttgaataatgcatggcttggtggcctgcaatattaaaatagaagtctgttgtgtgcttcatttcattggtgtgcccagtggcctcaatccagtgtcctattgggagacaatacacaccatccaccaagttgttttcattgtaagtacagcaacggtcatgatgaggtccattgccagaacgtgtccacgcggcccggctccgccccgtcctgcgccgcctcctcggccgccagctccacctccccgagccacaggcccggctcctgcagggccagggccccgtcgcccgccgcggtgccggccggcctcaggcggacggcaccgcgcggctcccaacgccccagctcgggccgcgaccccaccaccagcagctccggccgggcgccggccacggcgggtggcaccaccaccccaaagcggaagcgcatggcgggcggcggcggcgcgaat

SEQ ID NO: 18986 - RNA, 1397 nt, Homo sapiens
  source 1..1397: mol_type = other RNA
tggaggagaaggaaggtgatgccttggaacagactttaacaactgtgaggcaggataaaaaacaagtcctgaaagccatcactttttgaccatagtgagctcttcttttgtaacggttcaggcttctaaccttatttcctcctttggcaactgaccagctcacgcacacatactagtgatgaaatccacataactccatatcttttcctctacatggccaagagtttcagtgcaacaggaaagtgctgtcacggatccatcgtgcaacacatacagtgctgtaaagcaaaggcctcgtctgcctgcaggcagcaggaactgcacgcattacccttctgtctgatgtacagcctaactgcttcgtgcttcttctcatgtgttgagccacagctttcttgtagagtatttcaaaaatacagccccaaaacaaagcataatcgaaagtcatcccaggtgaaagtggttggcttgggggaggtcacacagtcctttcagttcaggtagaatccttgtttctaggtcatttgaccaacatcatcccaggctccttagggaaatcaggagggggcagaagcaggctgaccagctacaggctacacacagaagaacgaaccttcccaaatttctggaaaaaatcttcttgtgcccgggccaaggcctcttcgtcaatgtagacagccggcctcttggccatgaggaaatactgcaccttcctcagattccagcccatcacatactggagccagccgcagacagccgcggtggagcggcccaccccagcgttgcagtgcacgtacacgatgtgtcccttctccagcagcgcatgcagcaggcacaccgcctggggcagcatctgtactcggccttcggtgctcatatctggtgttggcatccagatgtaggccaagccttcttccctatatagtttaatcatagtgtctggagtcatgggctctgggtagcggttacagcctgaggaattctgtacaatatcccattcagtctggaaattcattacagctgtaatccccaattcatgcttcagtttgatggttacatgttccacctgacgagggcagctacccagccagatatttggtagaattcttgaataatgcatggcttggtggcctgcaatattaaaatagaagtctgttgtgtgcttcatttcattggtgtgcccagtggcctcaatccagtgtcctattgggagacaatacacaccatccaccaagttgttttcattgtaagtacagcaacggtcatgatgaggtccattgcctctagacagccgccttctaattgtgaaacgggggaagatcttggacctggtctctggagcgctccctatcttaaccaagtcacttactctagcaggtctcaggttctttgtctgt

SEQ ID NO: 18987 - RNA, 1859 nt, Homo sapiens
  source 1..1859: mol_type = other RNA
tggaggagaaggaaggtgatgccttggaacagactttaacaactgtgaggcaggataaaaaacaagtcctgaaagccatcactttttgaccatagtgagctcttcttttgtaacggttcaggcttctaaccttatttcctcctttggcaactgaccagctcacgcacacatactagtgatgaaatccacataactccatatcttttcctctacatggccaagagtttcagtgcaacaggaaagtgctgtcacggatccatcgtgcaacacatacagtgctgtaaagcaaaggcctcgtctgcctgcaggcagcaggaactgcacgcattacccttctgtctgatgtacagcctaactgcttcgtgcttcttctcatgtgttgagccacagctttcttgtagagtatttcaaaaatacagccccaaaacaaagcataatcgaaagtcatcccaggtgaaagtggttggcttgggggaggtcacacagtcctttcagttcaggtagaatccttgtttctaggtcatttgaccaacatcatcccaggctccttagggaaatcaggagggggcagaagcaggctgaccagctacaggctacacacagaagaacgaaccttcccaaatttctggaaaaaatcttcttgtgcccgggccaaggcctcttcgtcaatgtagacagccggcctcttggccatgaggaaatactgcaccttcctcagattccagcccatcacatactggagccagccgcagacagccgcggtggagcggcccaccccagcgttgcagtgcacgtacacgatgtgtcccttctccagcagcgcatgcagcaggcacaccgcctggggcagcatctgtactcggccttcggtgctcatatctggtgttggcatccagatgtaggccaagccttcttccctatatagtttaatcatagtgtctggagtcatgggctctgggtagcggttacagcctgaggaattctgtacaatatcccattcagtctggaaattcattacagctgtaatccccaattcatgcttcagtttgatggttacatgttccacctgacgagggcagctacccagccagatatttggtagaattcttgaataatgcatggcttggtggcctgcaatattaaaatagaagtctgttgtgtgcttcatttcattggtgtgcccagtggcctcaatccagtgtcctattgggagacaatacacaccatccaccaagttgttttcattgtaagtacagcaacggtcatgatgaggtccattgcctgtaatcccattactttgggtcacctaggcaggtggatcacttgtgcttcaggagttcgagacaggcctgggcaacatggcgaaaccccatttctactaaaaaatacaaaaattagctggccatggtgaaacatgcctgtggtttcagctactcagaaggttgacatgggaggatggcttgagcctgggaggcagaggctgcagtgagccaagatcatgccactgtactccagcctgggtgacagagccagacccttcccaggagagctctcctcccggctcccgcttcaggaacttgtaccagaacgtgtccacgcggcccggctccgccccgtcctgcgccgcctcctcggccgccagctccacctccccgagccacaggcccggctcctgcagggccagggccccgtcgcccgccgcggtgccggccggcctcaggcggacggcaccgcgcggctcccaacgccccagctcgggccgcgaccccaccaccagcagctccggccgggcgccggccacggcgggtggcaccaccaccccaaagcggaagcgcatggcgggcggcggcggcgcgaat

SEQ ID NO: 18988 - RNA, 1498 nt, Homo sapiens
  source 1..1498: mol_type = other RNA
tggaggagaaggaaggtgatgccttggaacagactttaacaactgtgaggcaggataaaaaacaagtcctgaaagccatcactttttgaccatagtgagctcttcttttgtaacggttcaggcttctaaccttatttcctcctttggcaactgaccagctcacgcacacatactagtgatgaaatccacataactccatatcttttcctctacatggccaagagtttcagtgcaacaggaaagtgctgtcacggatccatcgtgcaacacatacagtgctgtaaagcaaaggcctcgtctgcctgcaggcagcaggaactgcacgcattacccttctgtctgatgtacagcctaactgcttcgtgcttcttctcatgtgttgagccacagctttcttgtagagtatttcaaaaatacagccccaaaacaaagcataatcgaaagtcatcccaggtgaaagtggttggcttgggggaggtcacacagtcctttcagttcaggtagaatccttgtttctaggtcatttgaccaacatcatcccaggctccttagggaaatcaggagggggcagaagcaggctgaccagctacaggctacacacagaagaacgaaccttcccaaatttctggaaaaaatcttcttgtgcccgggccaaggcctcttcgtcaatgtagacagccggcctcttggccatgaggaaatactgcaccttcctcagattccagcccatcacatactggagccagccgcagacagccgcggtggagcggcccaccccagcgttgcagtgcacgtacacgatgtgtcccttctccagcagcgcatgcagcaggcacaccgcctggggcagcatctgtactcggccttcggtgctcatatctggtgttggcatccagatgtaggccaagccttcttccctatatagtttaatcatagtgtctggagtcatgggctctgggtagcggttacagcctgaggaattctgtacaatatcccattcagtctggaaattcattacagctgtaatccccaattcatgcttcagtttgatggttacatgttccacctgacgagggcagctacccagccagatatttggtagaattcttgaataatgcatggcttggtggcctgcaatattaaaatagaagtctgttgtgtgcttcatttcattggtgtgcccagtggcctcaatccagtgtcctattgggagacaatacacaccatccaccaagttgttttcattgtaagtacagcaacggtcatgatgaggtccattgcctgtgtgcaatacttaatgagagtgaccaccctctgtcgaaactctcctttgtaggttccgtaaaacttctttcttgaaagacagtattttatagcagttaagtgcatgggctcaagattcagactcagacttcattccaagttgtatgatttactctttgtaaacagtaatgagaaaatcatttaagcaaactgtgtctgttttcttatttgcaaa

SEQ ID NO: 18989 - RNA, 1604 nt, Homo sapiens
  source 1..1604: mol_type = other RNA
tggaggagaaggaaggtgatgccttggaacagactttaacaactgtgaggcaggataaaaaacaagtcctgaaagccatcactttttgaccatagtgagctcttcttttgtaacggttcaggcttctaaccttatttcctcctttggcaactgaccagctcacgcacacatactagtgatgaaatccacataactccatatcttttcctctacatggccaagagtttcagtgcaacaggaaagtgctgtcacggatccatcgtgcaacacatacagtgctgtaaagcaaaggcctcgtctgcctgcaggcagcaggaactgcacgcattacccttctgtctgatgtacagcctaactgcttcgtgcttcttctcatgtgttgagccacagctttcttgtagagtatttcaaaaatacagccccaaaacaaagcataatcgaaagtcatcccaggtgaaagtggttggcttgggggaggtcacacagtcctttcagttcaggtagaatccttgtttctaggtcatttgaccaacatcatcccaggctccttagggaaatcaggagggggcagaagcaggctgaccagctacaggctacacacagaagaacgaaccttcccaaatttctggaaaaaatcttcttgtgcccgggccaaggcctcttcgtcaatgtagacagccggcctcttggccatgaggaaatactgcaccttcctcagattccagcccatcacatactggagccagccgcagacagccgcggtggagcggcccaccccagcgttgcagtgcacgtacacgatgtgtcccttctccagcagcgcatgcagcaggcacaccgcctggggcagcatctgtactcggccttcggtgctcatatctggtgttggcatccagatgtaggccaagccttcttccctatatagtttaatcatagtgtctggagtcatgggctctgggtagcggttacagcctgaggaattctgtacaatatcccattcagtctggaaattcattacagctgtaatccccaattcatgcttcagtttgatggttacatgttccacctgacgagggcagctacccagccagatatttggtagaattcttgaataatgcatggcttggtggcctgcaatattaaaatagaagtctgttgtgtgcttcatttcattggtgtgcccagtggcctcaatccagtgtcctattgggagacaatacacaccatccaccaagttgttttcattgtaagtacagcaacggtcatgatgaggtccattgccttcccaggagagctctcctcccggctcccgcttcaggaacttgtaccagaacgtgtccacgcggcccggctccgccccgtcctgcgccgcctcctcggccgccagctccacctccccgagccacaggcccggctcctgcagggccagggccccgtcgcccgccgcggtgccggccggcctcaggcggacggcaccgcgcggctcccaacgccccagctcgggccgcgaccccaccaccagcagctccggccgggcgccggccacggcgggtggcaccaccaccccaaagcggaagcgcatggcgggcggcggcggcgcgaat

SEQ ID NO: 18990 - RNA, 1287 nt, Homo sapiens
  source 1..1287: mol_type = other RNA
tggaggagaaggaaggtgatgccttggaacagactttaacaactgtgaggcaggataaaaaacaagtcctgaaagccatcactttttgaccatagtgagctcttcttttgtaacggttcaggcttctaaccttatttcctcctttggcaactgaccagctcacgcacacatactagtgatgaaatccacataactccatatcttttcctctacatggccaagagtttcagtgcaacaggaaagtgctgtcacggatccatcgtgcaacacatacagtgctgtaaagcaaaggcctcgtctgcctgcaggcagcaggaactgcacgcattacccttctgtctgatgtacagcctaactgcttcgtgcttcttctcatgtgttgagccacagctttcttgtagagtatttcaaaaatacagccccaaaacaaagcataatcgaaagtcatcccaggtgaaagtggttggcttgggggaggtcacacagtcctttcagttcaggtagaatccttgtttctaggtcatttgaccaacatcatcccaggctccttagggaaatcaggagggggcagaagcaggctgaccagctacaggctacacacagaagaacgaaccttcccaaatttctggaaaaaatcttcttgtgcccgggccaaggcctcttcgtcaatgtagacagccggcctcttggccatgaggaaatactgcaccttcctcagattccagcccatcacatactggagccagccgcagacagccgcggtggagcggcccaccccagcgttgcagtgcacgtacacgatgtgtcccttctccagcagcgcatgcagcaggcacaccgcctggggcagcatctgtactcggccttcggtgctcatatctggtgttggcatccagatgtaggccaagccttcttccctatatagtttaatcatagtgtctggagtcatgggctctgggtagcggttacagcctgaggaattctgtacaatatcccattcagtctggaaattcattacagctgtaatccccaattcatgcttcagtttgatggttacatgttccacctgacgagggcagctacccagccagatatttggtagaattttattaaaaatcatttatatactggccataaaatatgtgtatttccaaatatagctgctgtagagctggactcttgagttgaatgtacgtcttgagctacaaaaatgagggaaagcaccatcttgaggcacaactggaattcaggcctttggtccctggatcagtaggggccaacagacac

SEQ ID NO: 18991 - RNA, 1532 nt, Homo sapiens
  source 1..1532: mol_type = other RNA
tggaggagaaggaaggtgatgccttggaacagactttaacaactgtgaggcaggataaaaaacaagtcctgaaagccatcactttttgaccatagtgagctcttcttttgtaacggttcaggcttctaaccttatttcctcctttggcaactgaccagctcacgcacacatactagtgatgaaatccacataactccatatcttttcctctacatggccaagagtttcagtgcaacaggaaagtgctgtcacggatccatcgtgcaacacatacagtgctgtaaagcaaaggcctcgtctgcctgcaggcagcaggaactgcacgcattacccttctgtctgatgtacagcctaactgcttcgtgcttcttctcatgtgttgagccacagctttcttgtagagtatttcaaaaatacagccccaaaacaaagcataatcgaaagtcatcccaggtgaaagtggttggcttgggggaggtcacacagtcctttcagttcaggtagaatccttgtttctaggtcatttgaccaacatcatcccaggctccttagggaaatcaggagggggcagaagcaggctgaccagctacaggctacacacagaagaacgaaccttcccaaatttctggaaaaaatcttcttgtgcccgggccaaggcctcttcgtcaatgtagacagccggcctcttggccatgaggaaatactgcaccttcctcagattccagcccatcacatactggagccagccgcagacagccgcggtggagcggcccaccccagcgttgcagtgcacgtacacgatgtgtcccttctccagcagcgcatgcagcaggcacaccgcctggggcagcatctgtactcggccttcggtgctcatatctggtgttggcatccagatgtaggccaagccttcttccctatatagtttaatcatagtgtctggagtcatgggctctgggtagcggttacagcctgaggaattctgtacaatatcccattcagtctggaaattcattacagctgtaatccccaattcatgcttcagtttgatggttacatgttccacctgacgagggcagctacccagccagatatttggtagaattttattaaaaatcatttatatactggccataaaatatgtgtatttccaaatatagctgctgtagagctggactcttgagttgaatgtacgtcttgagctacaaaaatgagggaaagcaccatcttgaggcacaactggaattcaggcctttggtccctggatctgaagttaagtagcaaattatgaacttaaagagatgaaagtggctgcctgtggaaagacaaaattgggggaggttgggtgggggaaagaagagggagaaagatttctttttctcataataaaacttgtagatctgataaattctttaaacacatgtttaaagaattggcatgtatgccttggctaaaaatcaaaaactaaaatgtaacacataaacctctctagataaatcataacatggaatgggtgctaatttctttttttt

SEQ ID NO: 18992 - RNA, 1476 nt, Homo sapiens
  source 1..1476: mol_type = other RNA
tggaggagaaggaaggtgatgccttggaacagactttaacaactgtgaggcaggataaaaaacaagtcctgaaagccatcactttttgaccatagtgagctcttcttttgtaacggttcaggcttctaaccttatttcctcctttggcaactgaccagctcacgcacacatactagtgatgaaatccacataactccatatcttttcctctacatggccaagagtttcagtgcaacaggaaagtgctgtcacggatccatcgtgcaacacatacagtgctgtaaagcaaaggcctcgtctgcctgcaggcagcaggaactgcacgcattacccttctgtctgatgtacagcctaactgcttcgtgcttcttctcatgtgttgagccacagctttcttgtagagtatttcaaaaatacagccccaaaacaaagcataatcgaaagtcatcccaggtgaaagtggttggcttgggggaggtcacacagtcctttcagttcaggtagaatccttgtttctaggtcatttgaccaacatcatcccaggctccttagggaaatcaggagggggcagaagcaggctgaccagctacaggctacacacagaagaacgaaccttcccaaatttctggaaaaaatcttcttgtgcccgggccaaggcctcttcgtcaatgtagacagccggcctcttggccatgaggaaatactgcaccttcctcagattccagcccatcacatactggagccagccgcagacagccgcggtggagcggcccaccccagcgttgcagtgcacgtacacgatgtgtcccttctccagcagcgcatgcagcaggcacaccgcctggggcagcatctgtactcggccttcggtgctcatatctggtgttggcatccagatgtaggccaagccttcttccctatatagtttaatcatagtgtctggagtcatgggctctgggtagcggttacagcctgaggaattctgtacaatatcccattcagtctggaaattcattacagctgtaatccccaattcatgcttcagtttgatggttacatgttccacctgacgagggcagctacccagccagatatttggtagaattttattaaaaatcatttatatactggccataaaatatgtgtatttccaaatatagctgctgtagagctggactcttgagttgaatgtacgtcttgagctacaaaaatgagggaaagcaccatcttgaggcacaactggaattcaggcctttggtccctggatcttgaataatgcatggcttggtggcctgcaatattaaaatagaagtctgttgtgtgcttcatttcattggtgtgcccagtggcctcaatccagtgtcctattgggagacaatacacaccatccaccaagttgttttcattgtaagtacagcaacggtcatgatgaggtccattgcagagattaactagcttgcccaaggtcacaaaact

SEQ ID NO: 18993 - RNA, 1765 nt, Homo sapiens
  source 1..1765: mol_type = other RNA
tggaggagaaggaaggtgatgccttggaacagactttaacaactgtgaggcaggataaaaaacaagtcctgaaagccatcactttttgaccatagtgagctcttcttttgtaacggttcaggcttctaaccttatttcctcctttggcaactgaccagctcacgcacacatactagtgatgaaatccacataactccatatcttttcctctacatggccaagagtttcagtgcaacaggaaagtgctgtcacggatccatcgtgcaacacatacagtgctgtaaagcaaaggcctcgtctgcctgcaggcagcaggaactgcacgcattacccttctgtctgatgtacagcctaactgcttcgtgcttcttctcatgtgttgagccacagctttcttgtagagtatttcaaaaatacagccccaaaacaaagcataatcgaaagtcatcccaggtgaaagtggttggcttgggggaggtcacacagtcctttcagttcaggtagaatccttgtttctaggtcatttgaccaacatcatcccaggctccttagggaaatcaggagggggcagaagcaggctgaccagctacaggctacacacagaagaacgaaccttcccaaatttctggaaaaaatcttcttgtgcccgggccaaggcctcttcgtcaatgtagacagccggcctcttggccatgaggaaatactgcaccttcctcagattccagcccatcacatactggagccagccgcagacagccgcggtggagcggcccaccccagcgttgcagtgcacgtacacgatgtgtcccttctccagcagcgcatgcagcaggcacaccgcctggggcagcatctgtactcggccttcggtgctcatatctggtgttggcatccagatgtaggccaagccttcttccctatatagtttaatcatagtgtctggagtcatgggctctgggtagcggttacagcctgaggaattctgtacaatatcccattcagtctggaaattcattacagctgtaatccccaattcatgcttcagtttgatggttacatgttccacctgacgagggcagctacccagccagatatttggtagaattttattaaaaatcatttatatactggccataaaatatgtgtatttccaaatatagctgctgtagagctggactcttgagttgaatgtacgtcttgagctacaaaaatgagggaaagcaccatcttgaggcacaactggaattcaggcctttggtccctggatcttgaataatgcatggcttggtggcctgcaatattaaaatagaagtctgttgtgtgcttcatttcattggtgtgcccagtggcctcaatccagtgtcctattgggagacaatacacaccatccaccaagttgttttcattgtaagtacagcaacggtcatgatgaggtccattgccttcccaggagagctctcctcccggctcccgcttcaggaacttgtaccagaacgtgtccacgcggcccggctccgccccgtcctgcgccgcctcctcggccgccagctccacctccccgagccacaggcccggctcctgcagggccagggccccgtcgcccgccgcggtgccggccggcctcaggcggacggcaccgcgcggctcccaacgccccagctcgggccgcgaccccaccaccagcagctccggccgggcgccggccacggcgggtggcaccaccaccccaaagcggaagcgcatggcgggcggcggcggcgcgaat

SEQ ID NO: 18994 - RNA, 1155 nt, Homo sapiens
  source 1..1155: mol_type = other RNA
tggaggagaaggaaggtgatgccttggaacagactttaacaactgtgaggcaggataaaaaacaagtcctgaaagccatcactttttgaccatagtgagctcttcttttgtaacggttcaggcttctaaccttatttcctcctttggcaactgaccagctcacgcacacatactagtgatgaaatccacataactccatatcttttcctctacatggccaagagtttcagtgcaacaggaaagtgctgtcacggatccatcgtgcaacacatacagtgctgtaaagcaaaggcctcgtctgcctgcaggcagcaggaactgcacgcattacccttctgtctgatgtacagcctaactgcttcgtgcttcttctcatgtgttgagccacagctttcttgtagagtatttcaaaaatacagccccaaaacaaagcataatcgaaagtcatcccaggtgaaagtggttggcttgggggaggtcacacagtcctttcagttcaggtagaatccttgtttctaggtcatttgaccaacatcatcccaggctccttagggaaatcaggagggggcagaagcaggctgaccagctacaggctacacacagaagaacgaaccttcccaaatttctggaaaaaatcttcttgtgcccgggccaaggcctcttcgtcaatgtagacagccggcctcttggccatgaggaaatactgcaccttcctcagattccagcccatcacatactggagccagccgcagacagccgcggtggagcggcccaccccagcgttgcagtgcacgtacacgatgtgtcccttctccagcagcgcatgcagcaggcacaccgcctggggcagcatctgtactcggccttgaataatgcatggcttggtggcctgcaatattaaaatagaagtctgttgtgtgcttcatttcattggtgtgcccagtggcctcaatccagtgtcctattgggagacaatacacaccatccaccaagttgttttcattgtaagtacagcaacggtcatgatgaggtccattgcctctagacagccgccttctaattgtgaaacgggggaagatcttggacctggtctctggagcgctccctatcttaaccaagtcacttactctagcaggtctcaggttctttgtctgt

SEQ ID NO: 18995 - RNA, 1362 nt, Homo sapiens
  source 1..1362: mol_type = other RNA
tggaggagaaggaaggtgatgccttggaacagactttaacaactgtgaggcaggataaaaaacaagtcctgaaagccatcactttttgaccatagtgagctcttcttttgtaacggttcaggcttctaaccttatttcctcctttggcaactgaccagctcacgcacacatactagtgatgaaatccacataactccatatcttttcctctacatggccaagagtttcagtgcaacaggaaagtgctgtcacggatccatcgtgcaacacatacagtgctgtaaagcaaaggcctcgtctgcctgcaggcagcaggaactgcacgcattacccttctgtctgatgtacagcctaactgcttcgtgcttcttctcatgtgttgagccacagctttcttgtagagtatttcaaaaatacagccccaaaacaaagcataatcgaaagtcatcccaggtgaaagtggttggcttgggggaggtcacacagtcctttcagttcaggtagaatccttgtttctaggtcatttgaccaacatcatcccaggctccttagggaaatcaggagggggcagaagcaggctgaccagctacaggctacacacagaagaacgaaccttcccaaatttctggaaaaaatcttcttgtgcccgggccaaggcctcttcgtcaatgtagacagccggcctcttggccatgaggaaatactgcaccttcctcagattccagcccatcacatactggagccagccgcagacagccgcggtggagcggcccaccccagcgttgcagtgcacgtacacgatgtgtcccttctccagcagcgcatgcagcaggcacaccgcctggggcagcatctgtactcggccttgaataatgcatggcttggtggcctgcaatattaaaatagaagtctgttgtgtgcttcatttcattggtgtgcccagtggcctcaatccagtgtcctattgggagacaatacacaccatccaccaagttgttttcattgtaagtacagcaacggtcatgatgaggtccattgccttcccaggagagctctcctcccggctcccgcttcaggaacttgtaccagaacgtgtccacgcggcccggctccgccccgtcctgcgccgcctcctcggccgccagctccacctccccgagccacaggcccggctcctgcagggccagggccccgtcgcccgccgcggtgccggccggcctcaggcggacggcaccgcgcggctcccaacgccccagctcgggccgcgaccccaccaccagcagctccggccgggcgccggccacggcgggtggcaccaccaccccaaagcggaagcgcatggcgggcggcggcggcgcgaat

SEQ ID NO: 18996 - RNA, 2127 nt, Homo sapiens
  source 1..2127: mol_type = other RNA
tggaggagaaggaaggtgatgggggaagagtgccagatgtgtctctcaacataggctattccagatgtggtccaccagcacgtggccttccagttgtgcctgaataacaccagatgtgatccaaggattaaatgtgaagggatgtgaaagtgctctggagcctgtaaactgttagcctgtctcccaaacgtaaggatggtgttagtattaatttgtctctgctgtatggccacaggcagctcttggccaacagcagtgtgagtgcctggtggtactggtcataagaaggcctgagtcacagcacgtggctggctcagcacacagtttactcatagaaaaccaggcaaaagcagatcagtaacatcactatggctgctgaaaggcagtgttgtcacaatgccatgaagacaaaaagttaagttgccattattaattaacatgagataatggcattaaaagataaatcttcaaggtcaaccaaggtttatagacatcaaaatctctgcactcctgccctgtcttctctaagtatcttctatactttcctgcttgagacttttgttttccctccatgtgctgggtgtcttaccccctttcctctgcttatctaaaagcctccatctctcagggcaggacaggacataaggtctctcactgagccttcgcctgaatgaagtgtgtgcttgtgcccacaattctactacacaggtgactttcctgtcttatgccaggtcagggaccaaccacattttgttctgatgcaggtgcagccaactcctcttgttggctttaagttctcagggttaattccatctttgtttagcatgttcattgtaattacatgggagagacttcagtttttgcatcaactttcagcgttttttttcttccttaaatatcacagttattccgtgtcaaaatttctcccaagtctattgtgaacatcactagcagttgtgctgtctgtgcaaagagtgagacggaacatgctgatgttgcagctgctgccatgtactcggctgctccagaaggttttacattttttaatgtaatgatagaggtttcagttacttacaggatgtaattttaaatatatatttgcaatagaaccagcttgatgtgcttacttttccattaatagaacactctgcactttttggaatgcatgtaccaaccttcccttaaagctcagctgaaactttaactccctattaggctttccaaccaatatctttctcctctaattttccttagttctgtctgctccactcatttaaggcctataatccctctcttattgtttctaaccgtttatgtgtcattacatgttccttgaaggaaagaagattcacctaccctttcttcttctacctaatacaaactactcacctcgcaaaacaatcaatagttatttgtatccaccttgtgtagcttagtgttcattgctggagtttgtgagggctgggggcctaatacacagtatctcacttcccagttagagtgatgaacatttagaaaagtaagacagggaggtgaagagataagagatgagttactaaagatgaagttggaagacacaactcagaacgaggcggttgggtgtcctcattgtccactgaactcagtggtggtaggtggtactcagtgagagctgcctcctgcagatggggagaaggctgaccccacggagtggtggagaaaggattatcatgtagacagctcactcccaaaggaagagggatagaggtattaaactcaatcatatccatttcaaatagaccaatccgaaaatcagtctagccgctttgaggcagagtgggtgaagggacagacagaagtcaggaggcttacacttctaagttccctctgcatgaaggccacatgagaactgctcctcctcaacaattatttttaaatagtcaaaaatctatcaaattttgaacacacctctttcaaaccttgctaactgccaacacaatcttctgaagttatccatcactcatgaaacaacaaaaacaaagaagaagagtgattttataacatcataaaatgctcgtgttactaaggatttgatatggtttggctgtgtccccacccaaatctcatcgtgaattgtagctcccataa

SEQ ID NO: 18997 - RNA, 210 nt, Homo sapiens
  source 1..210: mol_type = other RNA
tggagtccaggaatctgcattttaacaaactcactgggaaattctcgcgcacgccaaggtttcaaagaccagggtcccgtggcacagtgccgcacagttgtcaaaacaagtgctgtccaattgttttggttttaaattctcactgcgtcatgggaaatgtagtttcgagcctcctctctcccgacgccccagccaatcctccggcgcttt

SEQ ID NO: 18998 - RNA, 409 nt, Homo sapiens
  source 1..409: mol_type = other RNA
tggagtccaggaatctgcattttaacaagcatcagtgtgattctgataaagtttggagctgctggtcttaacttacagaattggatcctgcagtgtctctgaaaagaaaggtggggccagagagtggataagctctcaaaaataaaacttggtaatacaattgcaaatccttcaggaaaggaaagccctaaagatgccacagtcttatgtgcctgcaaagaaagctgctgagtttacactttttaaaaattctgtatcacttctccatcccactccccagaagataccactgttggtatttttagtatgtgtccttccagacttacttccatgcatatatggcttatatacatgtactcacaattcacacgcaagcttttttcattttctgatacatcatgaaaactca

SEQ ID NO: 18999 - RNA, 2318 nt, Homo sapiens
  source 1..2318: mol_type = other RNA
tggagtccaggaatctgcattttaacaagtcccctggtgcacaaggaaatttgagacccactgtgcccgacagcttgtgcacatggaaatttgttctgccaaagtttctcagataaaaacagagaggttctagccactgtcaggtcaaagctctggagagctgtgccatctcccaaagggagcagaacggtttgccatcaagccaggcaagagcccatttctgcctgtgcagctcgcagtctccgagcctgctgttgtttcatatcttgattgcttatcactcacccaaaataacctgaatgcaatcgcaccagctgcagctctctctgcaactcccttaatttagcagccaaacacattgggttccttcacagagcacaaggcctcagcacggggcccaggaaggggcccctccctcccagctgtctgtagtgagttgaatcatttccccctggaattcatgtccacctggaacctgagaatgtgactttatttggaactagagtatttgcaggtttaattaataaggatcaagataagatcacacaggattagggtgggccctaaatccaatgactgttgttaaaagaggagagaacagaagagacagagactggagtgatgcagcaataagctggggaatgccacggactgcccactgccgccacaagctaaaaagagccaaggaaggattcttccccagagccttcaaagggaccacagccctgccaacacctccatcccagatttccagcctccagaactgtaagggaatcaagttctgctgtttcaatccaccaggtttgtggtaattcgttagagcatccctaggaaaccaacacagcatcactgccataggcccccggcctggctcagcgcccactcagccccactctggcgggaaggaaagggccccacctgcaggcgattctccagatgggcagtttaacgtggcctgttaggatcagagctagtttctcccaaccgacatctttgaattctgcatctactaggcccatttcccacataaggagaaggacccttctgtcctctgcttgaaaggctgtattccaagaagggctgagtttggtagtgacaaatactggtccttgggcagtgtctggccggcggtgccatgcaagatgagtccctacagcttcatgccactccggcgccgtgagtccttccgggcaatggggctgaagttcacaatctccttgtagatgtgctgcttccattcatccactgtgagtttctcgtgttctaaggaatcatcaaacggctgctgggcctccgtctcttcctcagggtcccggaagggttcaaagaagggatgggtgagggcctgcgcggccgtcaggcgcttgtccacgtctagctccagcatcttctccagcaggtccgcagcctgggggctggcccgtgggaacagctgagtgaaatccttcctgggggtctgtggcagggactggatgtaggatttggccgctttgtcgttcagcttctgcacaaactccgtgccaggcaccccggtcactttcaggatctgggtcagctggtccaggtaatctttccccttgaacagagttttccctgtcagcatctctgccatgatacagcccacagaccagatgtccactgtctggttgtagtgcatccagctgaggatcacctcgggggctcggtaccagcgggtcaccacgtagccagtcatctcggcgtctgcatgtcgcgccagcccaaaatccagaatcttcagttcacagtcctcattcacagccaggttgcctggcttcaggtccctgtgcacgaccccagcagagtggatgtacttaaggcctttgagcatctgatacaccaggtactggatcttctcctcactgaactccatccccatgatcttctgcagatccgtctgcatgaagggcatcaccaggtagaagtcatagaagttgcgcagggaggaggctggggtgaagacatccaggagcccaatgacgttctcatgctgcatgtgcttcagcagcagcagctcccggtaggcgcgcttggcgaagatctcggactgaaagggtcggctcagcttcttgatggccaccttctcccctgaccgcttgtcgatggccgagcacacggagccataggccccgctgccgacgtgcgtcggggacacgtaggtcttgggcagctcccaggctgtcttgttgacgtcctgcttgtagaagccctttttccggatgaggctcatcccgggcacccgatctcggcggccccagcgtggcggctgcgttcgcggcccaacgggctcccagcgcccc

SEQ ID NO: 19000 - RNA, 2497 nt, Homo sapiens
  source 1..2497: mol_type = other RNA
tggagtccaggaatctgcattttaacaagtcccctggtgcacaaggaaatttgagacccactgtgcccgacagcttgtgcacatggaaatttgttctgccaaagtttctcagataaaaacagagaggttctagccactgtcaggtcaaagctctggagagctgtgccatctcccaaagggagcagaacggtttgccatcaagccaggcaagagcccatttctgcctgtgcagctcgcagtctccgagcctgctgttgtttcatatcttgattgcttatcactcacccaaaataacctgaatgcaatcgcaccagctgcagctctctctgcaactcccttaatttagcagccaaacacattgggttccttcacagagcacaaggcctcagcacggggcccaggaaggggcccctccctcccagctgtctgtagtgagttgaatcatttccccctggaattcatgtccacctggaacctgagaatgtgactttatttggaactagagtatttgcaggtttaattaataaggatcaagataagatcacacaggattagggtgggccctaaatccaatgactgttgttaaaagaggagagaacagaagagacagagactggagtgatgcagcaataagctggggaatgccacggactgcccactgccgccacaagctaaaaagagccaaggaaggattcttccccagagccttcaaagggaccacagccctgccaacacctccatcccagatttccagcctccagaactgtaagggaatcaagttctgctgtttcaatccaccaggtttgtggtaattcgttagagcatccctaggaaaccaacacagcatcactgccataggcccccggcctggctcagcgcccactcagccccactctggcgggaaggaaagggccccacctgcaggcgattctccagatgggcagtttaacgtggcctgttaggatcagagctagtttctcccaaccgacatctttgaattctgcatctactaggcccatttcccacataaggagaaggacccttctgtcctctgcttgaaaggctgtattccaagaagggctgagtttggtagtgacaaatactggtccttgggcagtgtctggccggcggtgccatgcaagatgagtccctacagcttcatgccactccggcgccgtgagtccttccgggcaatggggctgaagttcacaatctccttgtagatgtgctgcttccattcatccactgtgagtttctcgtgttctaaggaatcatcaaacggctgctgggcctccgtctcttcctcagggtcccggaagggttcaaagaagggatgggtgagggcctgcgcggccgtcaggcgcttgtccacgtctagctccagcatcttctccagcaggtccgcagcctgggggctggcccgtgggaacagctgagtgaaatccttcctgggggtctgtggcagggactggatgtaggatttggccgctttgtcgttcagcttctgcacaaactccgtgccaggcaccccggtcactttcaggatctgggtcagctggtccaggtaatctttccccttgaacagagttttccctgtcagcatctctgccatgatacagcccacagaccagatgtccactgtctggttgtagtgcatccagctgaggatcacctcgggggctcggtaccagcgggtcaccacgtagccagtcatctcggcgtctgcatgtcgcgccagcccaaaatccagaatcttcagttcacagtcctcattcacagccaggttgcctggcttcaggtccctgtgcacgaccccagcagagtggatgtacttaaggcctttgagcatctgatacaccaggtactggatcttctcctcactgaactccatccccatgatcttctgcagatccgtctgcatgaagggcatcaccaggtagaagtcatagaagttgcgcagggaggaggctggggtgaagacatccaggagcccaatgacgttctcatgctgcatgtgcttcagcagcagcagctcccggtaggcgcgcttggcgaagatctcggactgaaagggtcggctcagcttcttgatggccaccttctcccctgaccgcttgtcgatggccgagctagaatatgggggagccgcgggacgcagggcagggagtaggaagccaggcaggagctgagagaggggcacagcgccaggggcagcaacgtctcattgcgacgggatccacggcagggcgggagtctcactctgtctgcaacttggcgagccacctccccctcttggggcctcggtgtactcgtctgtaacagtgaggatctgcccgatgaactctggggtcttgcaagtgtacagtcctggagaaccaggcccagtcccaactcaacccccagagacctcactcagccactcggtgagaaaagggagatggccgctgggtggccccggggagggcgctgggccttgaggtccgcggtcaaggtggcg

SEQ ID NO: 19001 - RNA, 2166 nt, Homo sapiens
  source 1..2166: mol_type = other RNA
tggagtccaggaatctgcattttaacaagtcccctggtgcacaaggaaatttgagacccactgtgcccgacagcttgtgcacatggaaatttgttctgccaaagtttctcagataaaaacagagaggttctagccactgtcaggtcaaagctctggagagctgtgccatctcccaaagggagcagaacggtttgccatcaagccaggcaagagcccatttctgcctgtgcagctcgcagtctccgagcctgctgttgtttcatatcttgattgcttatcactcacccaaaataacctgaatgcaatcgcaccagctgcagctctctctgcaactcccttaatttagcagccaaacacattgggttccttcacagagcacaaggcctcagcacggggcccaggaaggggcccctccctcccagctgtctgtagtgagttgaatcatttccccctggaattcatgtccacctggaacctgagaatgtgactttatttggaactagagtatttgcaggtttaattaataaggatcaagataagatcacacaggattagggtgggccctaaatccaatgactgttgttaaaagaggagagaacagaagagacagagactggagtgatgcagcaataagctggggaatgccacggactgcccactgccgccacaagctaaaaagagccaaggaaggattcttccccagagccttcaaagggaccacagccctgccaacacctccatcccagatttccagcctccagaactgtaagggaatcaagttctgctgtttcaatccaccaggtttgtggtaattcgttagagcatccctaggaaaccaacacagcatcactgccataggcccccggcctggctcagcgcccactcagccccactctggcgggaaggaaagggccccacctgcaggcgattctccagatgggcagtttaacgtggcctgttaggatcagagctagtttctcccaaccgacatctttgaattctgcatctactaggcccatttcccacataaggagaaggacccttctgtcctctgcttgaaaggctgtattccaagaagggctgagtttggtagtgacaaatactggtccttgggcagtgtctggccggcggtgccatgcaagatgagtccctacagcttcatgccactccggcgccgtgagtccttccgggcaatggggctgaagttcacaatctccttgtagatgtgctgcttccattcatccactgtgagtttctcgtgttctaaggaatcatcaaacggctgctgggcctccgtctcttcctcagggtcccggaagggttcaaagaagggatgggtgagggcctgcgcggccgtcaggcgcttgtccacgtctagctccagcatcttctccagcaggtccgcagcctgggggctggcccgtgggaacagctgagtgaaatccttcctgggggtctgtggcagggactggatgtaggatttggcctgtctggttgtagtgcatccagctgaggatcacctcgggggctcggtaccagcgggtcaccacgtagccagtcatctcggcgtctgcatgtcgcgccagcccaaaatccagaatcttcagttcacagtcctcattcacagccaggttgcctggcttcaggtccctgtgcacgaccccagcagagtggatgtacttaaggcctttgagcatctgatacaccaggtactggatcttctcctcactgaactccatccccatgatcttctgcagatccgtctgcatgaagggcatcaccaggtagaagtcatagaagttgcgcagggaggaggctggggtgaagacatccaggagcccaatgacgttctcatgctgcatgtgcttcagcagcagcagctcccggtaggcgcgcttggcgaagatctcggactgaaagggtcggctcagcttcttgatggccaccttctcccctgaccgcttgtcgatggccgagcacacggagccataggccccgctgccgacgtgcgtcggggacacgtaggtcttgggcagctcccaggctgtcttgttgacgtcctgcttgtagaagccctttttccggatgaggctcatcccgggcacccgatctcggcggccccagcgtggcggctgcgttcgcggcccaacgggctcccagcgcccc

SEQ ID NO: 19002 - RNA, 622 nt, Homo sapiens
  source 1..622: mol_type = other RNA
tggagtccaggaatctgcattttaactagatttcttatgcttgttaaaaattgagaagcttaatctgggagaagagggactggcgaacagagagacagtgcaaattatttttatacattttagagatgatggggctatgggtgatttttatttgtgtgtgtgtatgtctgtttcagtattttccaaataaaacagtaagagaatgtctagagaggggctggagcaagatggccaaatataagtttccaccaatcatttcatcttcaggaataccgcatttaacaacaatctacaggaaaaaagcaccttcatacgaactaaaaatcaggtaagcatttacaatacctggttttaacttcatattgctgaaggacacactgaagagggtaggaggacagtctttagttgccaattcccgccatcctccatccctggcagtagctgcatggcacagagagaaggtttttccgcaagggtggggaaatagtctccaacatcatgaactgaagcatgcaagggccaccatccgagggcttcgagtctaagtctttgttcttcccgtgtcctctttcagtccagcctgtcccccttgcgcgggaaagtcctccatctctagttcccg

SEQ ID NO: 19003 - RNA, 2809 nt, Homo sapiens
  source 1..2809: mol_type = other RNA
tggagtccaggaatctgcattttaagaatattgtgcactgtgatttaaagccagaaaatgtgctgcttgcatcagcagagccatttcctcaggtgagatattctccagaaccttttaaatgattctggcaacattttcaaagcacccacataataaaaggcagtgtactaagtactgttggttaaaaatgcataccaccttacaaaaatagtttttagcctgtaactaccagtgaggattaataactaaatgaattcagatgttattagttatactgtttatattcaagattttttaagatttaactgcacatagattctgcaattcacctctccccaggggctgggaacgaagtgagcaagtatcaaccttggttggtgcatggtacttaggataaatacctcataaataaaacaaatggggtgttactggaaatgggagatagattttggttgaggcaggcagccacctcctttttctatgtagagtattgtattcaaacaacctacataaaataacatttctcatcaccacacatacacacaatggcatcgtgcttctgtgtcctggctacatgtagcactctctgatttttcttaattcagttgagttttttttttttccaagtgttcatcttgatccactaaatttattgcatgacctatgaaatggatcataacccaaattctgaaacaaccatcctgagaaataagtggtggtggtggtaccctgcagccattttccataattggcaaggatgattcctccgatcagctcaaatatctgttgccaaactattgtttatatacatttgaaacatgtacatttagacaaatggcaagactaaggacaacagataggtgttttcacttggtaaatataactcaaattgtcttttcaaataaaaagatatattaaaaatcgttcagcttttaaagtagtaatcatattctttttatgtttatgtggttaaaagtgattccctatcattttgaggtcgaaagggttgcctgatagttggtgcaatgttttaaataaactgcttccatatattatctcatttgatcttcaaaatagtagacaaaagatgcacactcctactggtaacattaaaactcccactttctgacctctattttagtgatccacagtgttccaatgagaagcaaagggaaaataatgtgatttacttgatacgctttttatgctcaagtgttagccatggctccacttctttaatcagttgccaaacttccaagtcatctttaccttatcaagatgttagctgaaatctggcatttaacaacaaaaaaagagtttgtatttcttcaggctcagtattcgtactcttcaaagacactgcagtatatgaaatgtgtttcctttattttgatttcttgggccgactgaagggtaaaatgtccaagctgaaatatcactgccaagcaagttcactaaacccagctacaacggatgcaaagggttttgactgacgtgcattcctctgatatcttccaccttgaagtctctgatgaggtagcaaggcaaaaaagttaaatctctctcccatcttctttggattcattaacatatcatatccttgaagtaactgctgcctcactgatggctcatttgatttatctaaaagaaccttcagccggacatcaatacccatattttttaaaaatgtgtgttgttttattgggcccagagaggctacttttccctgtgccattcttcgcaaataactgaagtccacatcagctgttagatctgctgttcctggggcaattaagacatcatgaagcttgtggtcgcaaaaccctctgaaggtatctgtctttgttccatcatgaccataatcagcaaccagtgcagcacctccagttaatgcaatgcgttgagaaagttcctcgatgataacaccagcatcaggacacacttcaacatgatcccttgtttcgtcatgttgtatgaaggcttctgctggggtggcagaaggtgccaaaacaaacctcagtttatcagaaacctgtggatcaatgtcaacaaatacttctcgccatccctgtggtgttttctgaaatttatgcacaggaagaacatcaaaaaattcatgtgcaagataaaagctgtacccttttggaacatcgtgcagatctcggtaccaggaaattggaatcccagacttagtgacacctttcatatacactggggatccagcatttcgctctaacgggaccttctctttagtcagtgtcaatgcttgaatctcacttaatttttggcttacctctaccagatgtactgaaatgtcacaatttttcagcacagatccaagttgagtgaacaccctcaaaatatctcccacgagggttcccctacctgggcccagttccaccagctggaaagctgtgctttttccagtggccatccattcactaatgaaccatatacctagtagctccccaaagatttgacttatttcaggtgaagtaatgaaatctcctttttcgcctagcatgtcacggtacacataataacccttggctggattagtcaacacctccttcatgtactcggccacagtgatgggaccagtagactttattttgtacataagatgccgcagcatcggcgtcaccgggttttctgcaggctcattcccggagctgaagtatttccctctccaaataaaaggaatggctgcgcgcgccacggcacacaacggccccaaacctgacctcagcagtacactcatgctgaaattcgcaggctagctcgctccgccaggagctggggcttagac

SEQ ID NO: 19004 - RNA, 3281 nt, Homo sapiens
  source 1..3281: mol_type = other RNA
tggagtccaggaatctgcattttaagaattccccaaaaatgccgctgaagtggttccagggcttgctttgagaatttccactctgagtctccctgctcctcacagctgagggttcctcatttctaggcttagccctacccctggctcccaggagcaattcacagagagtgagacaggcagtcacagacccaccagtgggggtcactaccagctgtgtcttcaccttggtacctgggtacagatgcctcccccaccaccaggcagagagcccaggagagcacgcccctgtgcctacgatgggccaggcatagcacaagtgctcagcaaacacagcagatgaacaaatgaagggacgccagctggaaccactgcctcccacaccagtcccgccaggcatccctcataaacgggctttcaccttgacacccagttgacttctacattctgcatccagggcctgccagctctggtgctgtgctgatggggaggagccctgtgcgtcccacacttgagctcctgtaatcccatggcggtgcccccagttcccgatgtgcctggctctacccccactttataaacgcagcaatcaagcagagccagaagtggcttcccaggccacacagccaggacatggaggggatgaaagctgtctccacccagccctccacccacctgaccagtctccaggtgacaccggccccagctgccaagtgccctccttgttcaagccaggctctgggaactggagagggacagaaggggtagggaacggtagggtgggccgggccagggcctgggttaggggggatgctggcctagagcggggcaggtgtggcctgtttctccctgaagagaggcccagcccctagcaggagaggggaagtgggagggcccagagaggaacccagtcctgaaatcaggacgcctgtgggggctttggaggcggggcagtcccaggagccacaagggcaggctgcaaccatgagcaagggtgtcgtagaattgtagagggacacagaaggcagtgtgtgggcggagctttcacaggacagtggaagcatctatgaggccaaggggcaggggtctgtgtccttggaggcatatgggagatgaggaactccttggatgttccagaagcttcacctgcaagaggaggagccggagcttctctctgctgtgcactccccagggacggctccgccactatcccgaggctgcccgtctacattccagctgtggacgctgctggctgggcctgagcagggtctcgggaactcagcaggcctgccgggtaaccctgggcctacccagatgcctgtgggatggggacttggtcctgaggaccctttacggacagcccactctgtgtctccgtgctgacctagcctggcacctggagtctcaggaggccaagggtgacccagagccctctttccctgtgcggccgtctcagggttgcagcaggatgcctcgtttcaagttgcagctcccctgccagctcgggtcagcctctcttgcattggaagcagctggggcatttccagagcatggaaaaaggcaggagccttttgcctcacttgtggaaaaacagattcagtgctggctggactggccaggtcagccagggtaccagccgcaggctccaggccatgaggctggacaatgcctggctggttggccagacagatgtggacggtgccagcacgtctgagaggcttcctaacttgggtcacgtcaggcagggcccccagggatgcctggggacaggccatgccaggcctgtgctggatgcacatcagacatcctggagctgaggttgacagcagctcaagggtgagtagggtcactgccccacggcggagatgaggaagctgaggttccaagagggggaagtgagaagtgtgggtgacagagctggtgataatggagctgggatcccactcagccttcccatctccccagcctgggacaggctgcctcctccaggctggccttggtggcagcagacctggctgctagccccccacagtgttgatcgtttcctgaacacgagtgacactgccttgttctctcccagccctggctccagcgtctgggcacagaaggcacagaacagacccagggtttcccagcgtgcgatgagctcaccactcactggtggcctgtgcttttggctggtacatggttgaacattttttcatagttgcacttttttaaagaaaatgtgtattagaaacattataaaactagcatatcacatctgtgattttatagctactattgtttaggatgaggctaagttttttaaaagtccattgattgaaaggaaaacatatgaaggaaatcatagcacaggaggtgcgtggctctagccaggctggagggaatgtggcttgggggagctggacagtccctgtggcctcctcagtgcttgtggaggctgccttgcacggtccccaggctttgaatgcagcatctcagactccactccgggactccccagtcccccaagccaagcaggaatgggaggcaggggagagcgctcccagcttagcttcggatacctgtcctggctctggccttcccagggagccctggcagggaagggacacagcccaggactagggtcatcctgggcagttttagttccagagcagcacagctcactgcctgacttgggggtaagcggcattcattgagataggggatgggggagctttgtcaatagggccacacttactgagccacgagggaggggtcaccgccccaggagagccagggctagaaggaatatacattagctgtgtgggcaggcagatccaaagcatgtgaagagcagggcttcccacgcctctgtcgtctctgatggccacctccgccaccaattgtctggctggaggggatgggatggaaggctgggaagtttaagtggggaaacaagagaagacaatgccaccacctggggaggaggggttgcctgccccagtgcccgtggcccaggaggacagcatgggataccaggttgagggaggtggtatggtggagatagaatgggctttggacccaagcctactttgggtatgacacttaacctctgtgagcctcagtttcctcatctataaaatgggcacagtaatatttcccaggatttttgagagaattaaatgatatgtgggtgcggtggaatactttctgatccatcaatctcttcttttttcttctcctgttttttttgtttgtttgtttgttttttgccttttctctctccttcctcctcagat

SEQ ID NO: 19005 - RNA, 2182 nt, Homo sapiens
  source 1..2182: mol_type = other RNA
tggagtccaggaatctgcattttacatatgcttctaggggatccttatgcccattaaagtttgcaaacctttatccgcccctctcaaaagtataccatcagtctaggggaagacagtcacatatgcggccaggaagaaagcaacagccctgttttggagaatgcttgcttctcccagacatatatgcatggggatgaggacccagagagtctctattgacttcaaggaaattaaccagtaactcaagcttggcttgtggctctgtaatggagagacggaggacaggtgaagaggctgtctctgaaatgagcatccccatctttccagggggcactggtatgcaggaaaaaaataacacataaaatggccagattttctacctatccttttttaagtggtgcaatcaccttttgtaagagtaaggggaacttttcttccttaatgggctaaagcatcatcaccctctcctatcctccatattcttccccttctcttaacttcctaattcctttggtggaggaggtggacaaacaagtagtcctcacaggaccaaaaccaagtttcgttttcagagtagatccaatttgaacatatcaagcacatcttccctagaagggcacagatgactggaaggcagatgtacatttctgaaaacacaaatgtcagaaccttccacccagggttggcccagcctgccatgtgaaggcaacacgagtgctatcacagatgcggcatcaggagtgtcagggtgagatcaggcatgcacatgaggtggaggaagacgagatttagagatgtccagcctttcgctggatttgagaattaacagcagactctctgtcttgccttagctctgaaggatacagcatcctttggtcactgtcagaggaagctcagttaccatcctcaaggatggtagaaaggctttccaaatccccctgggctaatccaggcagaggctggattctatcccgtccacctggaataatgcttccatcccccaaccctcatcatttgaaatttccaagaccaagataacgcatcctttcccagagacaaaggctttttgagatcatcatccatagagttctcagttagaaacaaaatgagacttgaaaggcaagttttaggattcagggttgaaccactgtcagcctggaggggacagttataaatagagggaggcgagtctcattccttcttggtgtgctctaggactcggtaggggaccccagaggcacttctggagccgtgctcttcttgcatgactggcagggtggcaggagcgtagatctcagaaatgttgtcattgttttccagagccccataggaaaaagaagctttaagttcaggctggacagtcatccctttatcgtgcatgttctgcatacctggcatggcatccatggaaatatagggctcaaatggaatgggcttcttcctgttacgcgtgattaagaagacgcccaagaatgcaatgaggcaccaagtaacgccaccaagagaagaatcacgacaatgttgttggcgttcttctccttgtagaagtagagcagcaagcagaacagaatgatctccaccagcatgtacaaaaggaaaggccagctcacgaggtgcctggtgacattctcgcctgtcatcttctcgtgactgttgggtgcgaatgtcaccagcaggtaggtacccacgacagccaaaccgcagccaacaaaggacaagacgtagcgcccttgtaggagaaggaggcctcgcttacggcgctggagctacttgtgggaggcagctgctgcagcttcagggctgcgctgtgggatccgtccatggtggtctagtggcgcatcccacagggcctggcctaggaggtggagctgctgctaggcggggcccaggccagatgccatctctccttgtggtgttcacctccctccagcagccgtcacttcctcatgacaaaagaatacttcaaggctgttttggcagatttacagccttctcctcagcttcactcagagaagtgccaatttccgtggctctcccaggcagacagagaggggtgtgttttccagttcttgcggtgctcggcggcgtctcctctaaggcccacctatcaaaaccttctgagaaatgactcggactcttcgtgcaacccggaggcacagcctccttcatcccttcccaattc

SEQ ID NO: 19006 - RNA, 2636 nt, Homo sapiens
  source 1..2636: mol_type = other RNA
tggagtccaggaatctgcattttacatatgcttctaggggatccttatgcccattaaagtttgcaaacctttatccgcccctctcaaaagtataccatcagtctaggggaagacagtcacatatgcggccaggaagaaagcaacagccctgttttggagaatgcttgcttctcccagacatatatgcatggggatgaggacccagagagtctctattgacttcaaggaaattaaccagtaactcaagcttggcttgtggctctgtaatggagagacggaggacaggtgaagaggctgtctctgaaatgagcatccccatctttccagggggcactggtatgcaggaaaaaaataacacataaaatggccagattttctacctatccttttttaagtggtgcaatcaccttttgtaagagtaaggggaacttttcttccttaatgggctaaagcatcatcaccctctcctatcctccatattcttccccttctcttaacttcctaattcctttggtggaggaggtggacaaacaagtagtcctcacaggaccaaaaccaagtttcgttttcagagtagatccaatttgaacatatcaagcacatcttccctagaagggcacagatgactggaaggcagatgtacatttctgaaaacacaaatgtcagaaccttccacccagggttggcccagcctgccatgtgaaggcaacacgagtgctatcacagatgcggcatcaggagtgtcagggtgagatcaggcatgcacatgaggtggaggaagacgagatttagagatgtccagcctttcgctggatttgagaattaacagcagactctctgtcttgccttagctctgaaggatacagcatcctttggtcactgtcagaggaagctcagttaccatcctcaaggatggtagaaaggctttccaaatccccctgggctaatccaggcagaggctggattctatcccgtccacctggaataatgcttccatcccccaaccctcatcatttgaaatttccaagaccaagataacgcatcctttcccagagacaaaggctttttgagatcatcatccatagagttctcagttagaaacaaaatgagacttgaaaggcaagttttaggattcagggttgaaccactgtcagcctggaggggacagttataaatagagggaggcgagtctcattccttcttggtgtgctctaggactcggtaggggaccccagaggcacttctggagccgtgctcttcttgcatgactggcagggtggcaggagcgtagatctcagaaatgttgtcattgttttccagagccccataggaaaaagaagctttaagttcaggctggacagtcatccctttatcgtgcatgttctgcatacctggcatggcatccatggaaatatagggctcaaatggaatgggcttcttcctgttacgcgtgattaagaagacgcccaagaatgcaatgaggcaccccagtgcaaacatgcagatgtgcagcacgtcctccccgatgaagtccaggtaaaatattgcacctgctgtgatagcaatggttgtggacagaatgtagcccacactggcaatcaaagaggagtcgtacatctgtgaggcttgactcaaaaaccaagtaacgccaccaagagaagaatcacgacaatgttgttggcgttcttctccttgtagaagtagagcagcaagcagaacagaatgatctccaccagcatgtacaaaaggaaaggccagctcacgaggtgcctggtgacattctcgcctgtcatcttctcgtgactgttgggtgcgaatgtcaccagcaggtaggtacccacgacagccaaaccgcagccaacaaaggacaagacgtagcgcctcagaaagtctttcggtttccacttttccttgatgaatatgattcctatgatggcactagctatcacagaaactgcgctgaggggcacgatgagtgacagcggcgcgaaggcgtaggaggcgaacacacccagctcgcccagaagcatcaggaacaggcccagccaccatgtcttggtcttgaaataggcccggggatccttggagcctgccaggcggatgtggcagtacttctggaggttaagtgcaatgctgaccacgaggtgcccgaagatcgccaagagggcgccaatcaggttttccttgtaggagaaggaggcctcgcttacggcgctggagctacttgtgggaggcagctgctgcagcttcagggctgcgctgtgggatccgtccatggtggtctagtggcgcatcccacagggcctggcctaggaggtggagctgctgctaggcggggcccaggccagatgccatctctccttgtggtgttcacctccctccagcagccgtcacttcctcatgacaaaagaatacttcaaggctgttttggcagatttacagccttctcctcagcttcactcagagaagtgccaatttccgtggctctcccaggcagacagagaggggtgtgttttccagttcttgcggtgctcggcggcgtctcctctaaggcccacctatcaaaaccttctgagaaatgactcggactcttcgtgcaacccggaggcacagcctccttcatcccttcccaattc

SEQ ID NO: 19007 - RNA, 2471 nt, Homo sapiens
  source 1..2471: mol_type = other RNA
tggagtccaggaatctgcattttacatatgcttctaggggatccttatgcccattaaagtttgcaaacctttatccgcccctctcaaaagtataccatcagtctaggggaagacagtcacatatgcggccaggaagaaagcaacagccctgttttggagaatgcttgcttctcccagacatatatgcatggggatgaggacccagagagtctctattgacttcaaggaaattaaccagtaactcaagcttggcttgtggctctgtaatggagagacggaggacaggtgaagaggctgtctctgaaatgagcatccccatctttccagggggcactggtatgcaggaaaaaaataacacataaaatggccagattttctacctatccttttttaagtggtgcaatcaccttttgtaagagtaaggggaacttttcttccttaatgggctaaagcatcatcaccctctcctatcctccatattcttccccttctcttaacttcctaattcctttggtggaggaggtggacaaacaagtagtcctcacaggaccaaaaccaagtttcgttttcagagtagatccaatttgaacatatcaagcacatcttccctagaagggcacagatgactggaaggcagatgtacatttctgaaaacacaaatgtcagaaccttccacccagggttggcccagcctgccatgtgaaggcaacacgagtgctatcacagatgcggcatcaggagtgtcagggtgagatcaggcatgcacatgaggtggaggaagacgagatttagagatgtccagcctttcgctggatttgagaattaacagcagactctctgtcttgccttagctctgaaggatacagcatcctttggtcactgtcagaggaagctcagttaccatcctcaaggatggtagaaaggctttccaaatccccctgggctaatccaggcagaggctggattctatcccgtccacctggaataatgcttccatcccccaaccctcatcatttgaaatttccaagaccaagataacgcatcctttcccagagacaaaggctttttgagatcatcatccatagagttctcagttagaaacaaaatgagacttgaaaggcaagttttaggattcagggttgaaccactgtcagcctggaggggacagttataaatagagggaggcgagtctcattccttcttggtgtgctctaggactcggtaggggaccccagaggcacttctggagccgtgctcttcttgcatgactggcagggtggcaggagcgtagatctcagaaatgttgtcattgttttccagagccccataggaaaaagaagctttaagttcaggctggacagtcatccctttatcgtgcatgttctgcatacctggcatggcatccatggaaatatagggctcaaatggaatgggcttcttcctgttacgcgtgattaagaagacgcccaagaatgcaatgaggcaccccagtgcaaacatgcagatgtgcagcacgtcctccccgatgaagtccaggtaaaatattgcacctgctgtgatagcaatggttgtggacagaatgtagcccacactggcaatcaaagaggagtcgtacatctgtgaggcttgactcaaaaacgcagcctgatagacggcggttgccaccatgcacacgaacatcacgtagaagatggggtagtcaagctgcaggttcccttgaatggacaagacaagcatcccagccacggccttgactgtcaccactgtcatggagccaagtaacgccaccaagagaagaatcacgacaatgttgttggcgttcttctccttgtagaagtagagcagcaagcagaacagaatgatctccaccagcatgtacaaaaggaaaggccagctcacgaggtgcctggtgacattctcgcctgtcatcttctcgtgactgttgggtgcgaatgtcaccagcaggtaggtacccacgacagccaaaccgcagccaacaaaggacaagacgtagcgcccttgtaggagaaggaggcctcgcttacggcgctggagctacttgtgggaggcagctgctgcagcttcagggctgcgctgtgggatccgtccatggtggtctagtggcgcatcccacagggcctggcctaggaggtggagctgctgctaggcggggcccaggccagatgccatctctccttgtggtgttcacctccctccagcagccgtcacttcctcatgacaaaagaatacttcaaggctgttttggcagatttacagccttctcctcagcttcactcagagaagtgccaatttccgtggctctcccaggcagacagagaggggtgtgttttccagttcttgcggtgctcggcggcgtctcctctaaggcccacctatcaaaaccttctgagaaatgactcggactcttcgtgcaacccggaggcacagcctccttcatcccttcccaattc

SEQ ID NO: 19008 - RNA, 2181 nt, Homo sapiens
  source 1..2181: mol_type = other RNA
tggagtccaggaatctgcattttacatatgcttctaggggatccttatgcccattaaagtttgcaaacctttatccgcccctctcaaaagtataccatcagtctaggggaagacagtcacatatgcggccaggaagaaagcaacagccctgttttggagaatgcttgcttctcccagacatatatgcatggggatgaggacccagagagtctctattgacttcaaggaaattaaccagtaactcaagcttggcttgtggctctgtaatggagagacggaggacaggtgaagaggctgtctctgaaatgagcatccccatctttccagggggcactggtatgcaggaaaaaaataacacataaaatggccagattttctacctatccttttttaagtggtgcaatcaccttttgtaagagtaaggggaacttttcttccttaatgggctaaagcatcatcaccctctcctatcctccatattcttccccttctcttaacttcctaattcctttggtggaggaggtggacaaacaagtagtcctcacaggaccaaaaccaagtttcgttttcagagtagatccaatttgaacatatcaagcacatcttccctagaagggcacagatgactggaaggcagatgtacatttctgaaaacacaaatgtcagaaccttccacccagggttggcccagcctgccatgtgaaggcaacacgagtgctatcacagatgcggcatcaggagtgtcagggtgagatcaggcatgcacatgaggtggaggaagacgagatttagagatgtccagcctttcgctggatttgagaattaacagcagactctctgtcttgccttagctctgaaggatacagcatcctttggtcactgtcagaggaagctcagttaccatcctcaaggatggtagaaaggctttccaaatccccctgggctaatccaggcagaggctggattctatcccgtccacctggaataatgcttccatcccccaaccctcatcatttgaaatttccaagaccaagataacgcatcctttcccagagacaaaggctttttgagatcatcatccatagagttctcagttagaaacaaaatgagacttgaaaggcaagttttaggattcagggttgaaccactgtcagcctggaggggacagttataaatagagggaggcgagtctcattccttcttggtgtgctctaggactcggtaggggaccccagaggcacttctggagccgtgctcttcttgcatgactggcagggtggcaggagcgtagatctcagaaatgttgtcattgttttccagagccccataggaaaaagaagctttaagttcaggctggacagtcatccctttatcgtgcatgttctgcatacctggcatggcatccatggaaatatagggctcaaatggaatgggcttcttcctgttacgcgtgattaagaagacgcccaagaatgcaatgaggcaccccagtgcaaacatgcagatgtgcagcacgtcctccccgatgaagtccaggtaaaatattgcacctgctgtgatagcaatggttgtggacagaatgtagcccacactggcaatcaaagaggagtcgtacatctgtgaggcttgactcaaaaacgcagcctgatagacggcggttgccaccatgcacacgaacatcacgtagaagatggggtagtcaagctgcaggttcccttgaatggacaagacaagcatcccagccacggccttgactgtcaccactgtcatggagccaagtaacgccaccaagagaagaatcacgacaatgttgttggcgttcttctccttgtagaagtagagcagcaagcagaacagaatgatctccaccagcatgtacaaaaggaaaggccagctcacgaggtgcctggtgacattctcgcctgtcatcttctcgtgactgttgggtgcgaatgtcaccagcaggtaggtacccacgacagccaaaccgcagccaacaaaggacaagacgtagcgcctcagaaagtctttcggtttccacttttccttgatgaatatgattcctatgatggcactagcggcggcgtctcctctaaggcccacctatcaaaaccttctgagaaatgactcggactcttcgtgcaacccggaggcacagcctccttcatcccttcccaattc

SEQ ID NO: 19009 - RNA, 2422 nt, Homo sapiens
  source 1..2422: mol_type = other RNA
tggagtccaggaatctgcattttacatatgcttctaggggatccttatgcccattaaagtttgcaaacctttatccgcccctctcaaaagtataccatcagtctaggggaagacagtcacatatgcggccaggaagaaagcaacagccctgttttggagaatgcttgcttctcccagacatatatgcatggggatgaggacccagagagtctctattgacttcaaggaaattaaccagtaactcaagcttggcttgtggctctgtaatggagagacggaggacaggtgaagaggctgtctctgaaatgagcatccccatctttccagggggcactggtatgcaggaaaaaaataacacataaaatggccagattttctacctatccttttttaagtggtgcaatcaccttttgtaagagtaaggggaacttttcttccttaatgggctaaagcatcatcaccctctcctatcctccatattcttccccttctcttaacttcctaattcctttggtggaggaggtggacaaacaagtagtcctcacaggaccaaaaccaagtttcgttttcagagtagatccaatttgaacatatcaagcacatcttccctagaagggcacagatgactggaaggcagatgtacatttctgaaaacacaaatgtcagaaccttccacccagggttggcccagcctgccatgtgaaggcaacacgagtgctatcacagatgcggcatcaggagtgtcagggtgagatcaggcatgcacatgaggtggaggaagacgagatttagagatgtccagcctttcgctggatttgagaattaacagcagactctctgtcttgccttagctctgaaggatacagcatcctttggtcactgtcagaggaagctcagttaccatcctcaaggatggtagaaaggctttccaaatccccctgggctaatccaggcagaggctggattctatcccgtccacctggaataatgcttccatcccccaaccctcatcatttgaaatttccaagaccaagataacgcatcctttcccagagacaaaggctttttgagatcatcatccatagagttctcagttagaaacaaaatgagacttgaaaggcaagttttaggattcagggttgaaccactgtcagcctggaggggacagttataaatagagggaggcgagtctcattccttcttggtgtgctctaggactcggtaggggaccccagaggcacttctggagccgtgctcttcttgcatgactggcagggtggcaggagcgtagatctcagaaatgttgtcattgttttccagagccccataggaaaaagaagctttaagttcaggctggacagtcatccctttatcgtgcatgttctgcatacctggcatggcatccatggaaatatagggctcaaatggaatgggcttcttcctgttacgcgtgattaagaagacgcccaagaatgcaatgaggcaccccagtgcaaacatgcagatgtgcagcacgtcctccccgatgaagtccaggtaaaatattgcacctgctgtgatagcaatggttgtggacagaatgtagcccacactggcaatcaaagaggagtcgtacatctgtgaggcttgactcaaaaacgcagcctgatagacggcggttgccaccatgcacacgaacatcacgtagaagatggggtagtcaagctgcaggttcccttgaatggacaagacaagcatcccagccacggccttgactgtcaccactgtcatggagccaagtaacgccaccaagagaagaatcacgacaatgttgttggcgttcttctccttgtagaagtagagcagcaagcagaacagaatgatctccaccagcatgtacaaaaggaaaggccagctcacgaggtgcctggtgacattctcgcctgtcatcttctcgtgactgttgggtgcgaatgtcaccagcaggtaggtacccacgacagccaaaccgcagccaacaaaggacaagacgtagcgcctcagaaagtctttcggtttccacttttccttgatgaatatgattcctatgatggcactagctatcacagaaactgcgctgaggggcacgatgagtgacagcggcgcgaaggcgtaggaggcgaacacacccagctcgcccagaagcatcaggaacaggcccagccaccatgtcttggtcttgaaataggcccggggatccttggagcctgccaggcggatgtggcagtacttctggaggttaagtgcaatgctgaccacgaggtgcccgaagatcgccaagagggcgccaatcaggttttccggcggcgtctcctctaaggcccacctatcaaaaccttctgagaaatgactcggactcttcgtgcaacccggaggcacagcctccttcatcccttcccaattc

SEQ ID NO: 19010 - RNA, 2734 nt, Homo sapiens
  source 1..2734: mol_type = other RNA
tggagtccaggaatctgcattttacatatgcttctaggggatccttatgcccattaaagtttgcaaacctttatccgcccctctcaaaagtataccatcagtctaggggaagacagtcacatatgcggccaggaagaaagcaacagccctgttttggagaatgcttgcttctcccagacatatatgcatggggatgaggacccagagagtctctattgacttcaaggaaattaaccagtaactcaagcttggcttgtggctctgtaatggagagacggaggacaggtgaagaggctgtctctgaaatgagcatccccatctttccagggggcactggtatgcaggaaaaaaataacacataaaatggccagattttctacctatccttttttaagtggtgcaatcaccttttgtaagagtaaggggaacttttcttccttaatgggctaaagcatcatcaccctctcctatcctccatattcttccccttctcttaacttcctaattcctttggtggaggaggtggacaaacaagtagtcctcacaggaccaaaaccaagtttcgttttcagagtagatccaatttgaacatatcaagcacatcttccctagaagggcacagatgactggaaggcagatgtacatttctgaaaacacaaatgtcagaaccttccacccagggttggcccagcctgccatgtgaaggcaacacgagtgctatcacagatgcggcatcaggagtgtcagggtgagatcaggcatgcacatgaggtggaggaagacgagatttagagatgtccagcctttcgctggatttgagaattaacagcagactctctgtcttgccttagctctgaaggatacagcatcctttggtcactgtcagaggaagctcagttaccatcctcaaggatggtagaaaggctttccaaatccccctgggctaatccaggcagaggctggattctatcccgtccacctggaataatgcttccatcccccaaccctcatcatttgaaatttccaagaccaagataacgcatcctttcccagagacaaaggctttttgagatcatcatccatagagttctcagttagaaacaaaatgagacttgaaaggcaagttttaggattcagggttgaaccactgtcagcctggaggggacagttataaatagagggaggcgagtctcattccttcttggtgtgctctaggactcggtaggggaccccagaggcacttctggagccgtgctcttcttgcatgactggcagggtggcaggagcgtagatctcagaaatgttgtcattgttttccagagccccataggaaaaagaagctttaagttcaggctggacagtcatccctttatcgtgcatgttctgcatacctggcatggcatccatggaaatatagggctcaaatggaatgggcttcttcctgttacgcgtgattaagaagacgcccaagaatgcaatgaggcaccccagtgcaaacatgcagatgtgcagcacgtcctccccgatgaagtccaggtaaaatattgcacctgctgtgatagcaatggttgtggacagaatgtagcccacactggcaatcaaagaggagtcgtacatctgtgaggcttgactcaaaaacgcagcctgatagacggcggttgccaccatgcacacgaacatcacgtagaagatggggtagtcaagctgcaggttcccttgaatggacaagacaagcatcccagccacggccttgactgtcaccactgtcatggagccaagtaacgccaccaagagaagaatcacgacaatgttgttggcgttcttctccttgtagaagtagagcagcaagcagaacagaatgatctccaccagcatgtacaaaaggaaaggccagctcacgaggtgcctggtgacattctcgcctgtcatcttctcgtgactgttgggtgcgaatgtcaccagcaggtaggtacccacgacagccaaaccgcagccaacaaaggacaagacgtagcgcctcagaaagtctttcggtttccacttttccttgatgaatatgattcctatgatggcactagctatcacagaaactgcgctgaggggcacgatgagtgacagcggcgcgaaggcgtaggaggcgaacacacccagctcgcccagaagcatcaggaacaggcccagccaccatgtcttggtcttgaaataggcccggggatccttggagcctgccaggcggatgtggcagtacttctggaggttaagtgcaatgctgaccacgaggtgcccgaagatcgccaagagggcgccaatcaggttttcctcgcggacggcggaaggtggactcgcgaatgttaggcctgtgggtgccatagcgaccgggaggttgggctggccagattcagctgccgggaccggaccaggtaggaagcagttccggcggggggaccggtccctgaggtcgtggggaagaggacacggcgcaccatgtcctccgcatgggacgcccgcggagaccccccggcctccgggtgcttgcggaattccagggctgagctaggtggagccccgagggcgggaagaagccaccatgggagttgcccctgcgtcggggcgtgtcctcggtgtttccacccgaaaagtggtgacaactggggcttgcctgctccaccgagctcctgccaggggcgtgggcgtccgacccttctggctcaggctccgcgagtgcgcaaaagtt

SEQ ID NO: 19011 - RNA, 2854 nt, Homo sapiens
  source 1..2854: mol_type = other RNA
tggagtccaggaatctgcattttacatatgcttctaggggatccttatgcccattaaagtttgcaaacctttatccgcccctctcaaaagtataccatcagtctaggggaagacagtcacatatgcggccaggaagaaagcaacagccctgttttggagaatgcttgcttctcccagacatatatgcatggggatgaggacccagagagtctctattgacttcaaggaaattaaccagtaactcaagcttggcttgtggctctgtaatggagagacggaggacaggtgaagaggctgtctctgaaatgagcatccccatctttccagggggcactggtatgcaggaaaaaaataacacataaaatggccagattttctacctatccttttttaagtggtgcaatcaccttttgtaagagtaaggggaacttttcttccttaatgggctaaagcatcatcaccctctcctatcctccatattcttccccttctcttaacttcctaattcctttggtggaggaggtggacaaacaagtagtcctcacaggaccaaaaccaagtttcgttttcagagtagatccaatttgaacatatcaagcacatcttccctagaagggcacagatgactggaaggcagatgtacatttctgaaaacacaaatgtcagaaccttccacccagggttggcccagcctgccatgtgaaggcaacacgagtgctatcacagatgcggcatcaggagtgtcagggtgagatcaggcatgcacatgaggtggaggaagacgagatttagagatgtccagcctttcgctggatttgagaattaacagcagactctctgtcttgccttagctctgaaggatacagcatcctttggtcactgtcagaggaagctcagttaccatcctcaaggatggtagaaaggctttccaaatccccctgggctaatccaggcagaggctggattctatcccgtccacctggaataatgcttccatcccccaaccctcatcatttgaaatttccaagaccaagataacgcatcctttcccagagacaaaggctttttgagatcatcatccatagagttctcagttagaaacaaaatgagacttgaaaggcaagttttaggattcagggttgaaccactgtcagcctggaggggacagttataaatagagggaggcgagtctcattccttcttggtgtgctctaggactcggtaggggaccccagaggcacttctggagccgtgctcttcttgcatgactggcagggtggcaggagcgtagatctcagaaatgttgtcattgttttccagagccccataggaaaaagaagctttaagttcaggctggacagtcatccctttatcgtgcatgttctgcatacctggcatggcatccatggaaatatagggctcaaatggaatgggcttcttcctgttacgcgtgattaagaagacgcccaagaatgcaatgaggcaccccagtgcaaacatgcagatgtgcagcacgtcctccccgatgaagtccaggtaaaatattgcacctgctgtgatagcaatggttgtggacagaatgtagcccacactggcaatcaaagaggagtcgtacatctgtgaggcttgactcaaaaacgcagcctgatagacggcggttgccaccatgcacacgaacatcacgtagaagatggggtagtcaagctgcaggttcccttgaatggacaagacaagcatcccagccacggccttgactgtcaccactgtcatggagccaagtaacgccaccaagagaagaatcacgacaatgttgttggcgttcttctccttgtagaagtagagcagcaagcagaacagaatgatctccaccagcatgtacaaaaggaaaggccagctcacgaggtgcctggtgacattctcgcctgtcatcttctcgtgactgttgggtgcgaatgtcaccagcaggtaggtacccacgacagccaaaccgcagccaacaaaggacaagacgtagcgcctcagaaagtctttcggtttccacttttccttgatgaatatgattcctatgatggcactagctatcacagaaactgcgctgaggggcacgatgagtgacagcggcgcgaaggcgtaggaggcgaacacacccagctcgcccagaagcatcaggaacaggcccagccaccatgtcttggtcttgaaataggcccggggatccttggagcctgccaggcggatgtggcagtacttctggaggttaagtgcaatgctgaccacgaggtgcccgaagatcgccaagagggcgccaatcaggttttcctgtaaggaaagttcacaggagtggacatgatttgggcacaagccagggggccccaggacacttctgacactcaaccatttgcttgtaggagaaggaggcctcgcttacggcgctggagctacttgtgggaggcagctgctgcagcttcagggctgcgctgtgggatccgtccatggtggtctagtggcgcatcccacagggcctggcctaggaggtggagctgctgctaggcggggcccaggccagatgccatctctccttgtggtgttcacctccctccagcagccgtcacttcctcatgacaaaagaatacttcaaggctgttttggcagatttacagccttctcctcagcttcactcagagaagtgccaatttccgtggctctcccaggcagacagagaggggtgtgttttccagttcttgcggtgctcggcggcgtctcctctaaggcccacctatcaaaaccttctgagaaatgactcggactcttcgtgcaacccggaggcacagcctccttcatcccttcccaattc

SEQ ID NO: 19012 - RNA, 2882 nt, Homo sapiens
  source 1..2882: mol_type = other RNA
tggagtccaggaatctgcattttacatatgcttctaggggatccttatgcccattaaagtttgcaaacctttatccgcccctctcaaaagtataccatcagtctaggggaagacagtcacatatgcggccaggaagaaagcaacagccctgttttggagaatgcttgcttctcccagacatatatgcatggggatgaggacccagagagtctctattgacttcaaggaaattaaccagtaactcaagcttggcttgtggctctgtaatggagagacggaggacaggtgaagaggctgtctctgaaatgagcatccccatctttccagggggcactggtatgcaggaaaaaaataacacataaaatggccagattttctacctatccttttttaagtggtgcaatcaccttttgtaagagtaaggggaacttttcttccttaatgggctaaagcatcatcaccctctcctatcctccatattcttccccttctcttaacttcctaattcctttggtggaggaggtggacaaacaagtagtcctcacaggaccaaaaccaagtttcgttttcagagtagatccaatttgaacatatcaagcacatcttccctagaagggcacagatgactggaaggcagatgtacatttctgaaaacacaaatgtcagaaccttccacccagggttggcccagcctgccatgtgaaggcaacacgagtgctatcacagatgcggcatcaggagtgtcagggtgagatcaggcatgcacatgaggtggaggaagacgagatttagagatgtccagcctttcgctggatttgagaattaacagcagactctctgtcttgccttagctctgaaggatacagcatcctttggtcactgtcagaggaagctcagttaccatcctcaaggatggtagaaaggctttccaaatccccctgggctaatccaggcagaggctggattctatcccgtccacctggaataatgcttccatcccccaaccctcatcatttgaaatttccaagaccaagataacgcatcctttcccagagacaaaggctttttgagatcatcatccatagagttctcagttagaaacaaaatgagacttgaaaggcaagttttaggattcagggttgaaccactgtcagcctggaggggacagttataaatagagggaggcgagtctcattccttcttggtgtgctctaggactcggtaggggaccccagaggcacttctggagccgtgctcttcttgcatgactggcagggtggcaggagcgtagatctcagaaatgttgtcattgttttccagagccccataggaaaaagaagctttaagttcaggctggacagtcatccctttatcgtgcatgttctgcatacctggcatggcatccatggaaatatagggctcaaatggaatgggcttcttcctgttacgcgtgattaagaagacgcccaagaatgcaatgaggcaccccagtgcaaacatgcagatgtgcagcacgtcctccccgatgaagtccaggtaaaatattgcacctgctgtgatagcaatggttgtggacagaatgtagcccacactggcaatcaaagaggagtcgtacatctgtgaggcttgactcaaaaacgcagcctgatagacggcggttgccaccatgcacacgaacatcacgtagaagatggggtagtcaagctgcaggttcccttgaatggacaagacaagcatcccagccacggccttgactgtcaccactgtcatggagccaagtaacgccaccaagagaagaatcacgacaatgttgttggcgttcttctccttgtagaagtagagcagcaagcagaacagaatgatctccaccagcatgtacaaaaggaaaggccagctcacgaggtgcctggtgacattctcgcctgtcatcttctcgtgactgttgggtgcgaatgtcaccagcaggtaggtacccacgacagccaaaccgcagccaacaaaggacaagacgtagcgcctcagaaagtctttcggtttccacttttccttgatgaatatgattcctatgatggcactagctatcacagaaactgcgctgaggggcacgatgagtgacagcggcgcgaaggcgtaggaggcgaacacacccagctcgcccagaagcatcaggaacaggcccagccaccatgtcttggtcttgaaataggcccggggatccttggagcctgccaggcggatgtggcagtacttctggaggttaagtgcaatgctgaccacgaggtgcccgaagatcgccaagagggcgccaatcaggttttccttgaatccagcctctgtccttcatgacactgtgactcggacatatctttgggcatttgtttcctcaactgtaaaatggagttattaacggtacttactcctcagggcagcttgtaggagaaggaggcctcgcttacggcgctggagctacttgtgggaggcagctgctgcagcttcagggctgcgctgtgggatccgtccatggtggtctagtggcgcatcccacagggcctggcctaggaggtggagctgctgctaggcggggcccaggccagatgccatctctccttgtggtgttcacctccctccagcagccgtcacttcctcatgacaaaagaatacttcaaggctgttttggcagatttacagccttctcctcagcttcactcagagaagtgccaatttccgtggctctcccaggcagacagagaggggtgtgttttccagttcttgcggtgctcggcggcgtctcctctaaggcccacctatcaaaaccttctgagaaatgactcggactcttcgtgcaacccggaggcacagcctccttcatcccttcccaattc

SEQ ID NO: 19013 - RNA, 3004 nt, Homo sapiens
  source 1..3004: mol_type = other RNA
tggagtccaggaatctgcattttacatatgcttctaggggatccttatgcccattaaagtttgcaaacctttatccgcccctctcaaaagtataccatcagtctaggggaagacagtcacatatgcggccaggaagaaagcaacagccctgttttggagaatgcttgcttctcccagacatatatgcatggggatgaggacccagagagtctctattgacttcaaggaaattaaccagtaactcaagcttggcttgtggctctgtaatggagagacggaggacaggtgaagaggctgtctctgaaatgagcatccccatctttccagggggcactggtatgcaggaaaaaaataacacataaaatggccagattttctacctatccttttttaagtggtgcaatcaccttttgtaagagtaaggggaacttttcttccttaatgggctaaagcatcatcaccctctcctatcctccatattcttccccttctcttaacttcctaattcctttggtggaggaggtggacaaacaagtagtcctcacaggaccaaaaccaagtttcgttttcagagtagatccaatttgaacatatcaagcacatcttccctagaagggcacagatgactggaaggcagatgtacatttctgaaaacacaaatgtcagaaccttccacccagggttggcccagcctgccatgtgaaggcaacacgagtgctatcacagatgcggcatcaggagtgtcagggtgagatcaggcatgcacatgaggtggaggaagacgagatttagagatgtccagcctttcgctggatttgagaattaacagcagactctctgtcttgccttagctctgaaggatacagcatcctttggtcactgtcagaggaagctcagttaccatcctcaaggatggtagaaaggctttccaaatccccctgggctaatccaggcagaggctggattctatcccgtccacctggaataatgcttccatcccccaaccctcatcatttgaaatttccaagaccaagataacgcatcctttcccagagacaaaggctttttgagatcatcatccatagagttctcagttagaaacaaaatgagacttgaaaggcaagttttaggattcagggttgaaccactgtcagcctggaggggacagttataaatagagggaggcgagtctcattccttcttggtgtgctctaggactcggtaggggaccccagaggcacttctggagccgtgctcttcttgcatgactggcagggtggcaggagcgtagatctcagaaatgttgtcattgttttccagagccccataggaaaaagaagctttaagttcaggctggacagtcatccctttatcgtgcatgttctgcatacctggcatggcatccatggaaatatagggctcaaatggaatgggcttcttcctgttacgcgtgattaagaagacgcccaagaatgcaatgaggcaccccagtgcaaacatgcagatgtgcagcacgtcctccccgatgaagtccaggtaaaatattgcacctgctgtgatagcaatggttgtggacagaatgtagcccacactggcaatcaaagaggagtcgtacatctgtgaggcttgactcaaaaacgcagcctgatagacggcggttgccaccatgcacacgaacatcacgtagaagatggggtagtcaagctgcaggttcccttgaatggacaagacaagcatcccagccacggccttgactgtcaccactgtcatggagccaagtaacgccaccaagagaagaatcacgacaatgttgttggcgttcttctccttgtagaagtagagcagcaagcagaacagaatgatctccaccagcatgtacaaaaggaaaggccagctcacgaggtgcctggtgacattctcgcctgtcatcttctcgtgactgttgggtgcgaatgtcaccagcaggtaggtacccacgacagccaaaccgcagccaacaaaggacaagacgtagcgcctcagaaagtctttcggtttccacttttccttgatgaatatgattcctatgatggcactagctatcacagaaactgcgctgaggggcacgatgagtgacagcggcgcgaaggcgtaggaggcgaacacacccagctcgcccagaagcatcaggaacaggcccagccaccatgtcttggtcttgaaataggcccggggatccttggagcctgccaggcggatgtggcagtacttctggaggttaagtgcaatgctgaccacgaggtgcccgaagatcgccaagagggcgccaatcaggttttccttgtaggagaaggaggcctcgcttacggcgctggagctacttgtgggaggcagctgctgcagcttcagggctgcgctgtgggatccgtccatggtggtctagtggcgcatcccacagggcctggcctaggaggtggagctgctgctaggcggggcccaggccagatgccatctctccttgtggtgttcacctccctccagcagccgtcacttcctcatgacaaaagaatacttcaaggctgttttggcagatttacagccttctcctcagcttcactcagagaagtgccaatttccgtggctctcccaggcagacagagaggggtgtgttttccagttcttgcggtgctaactcgaggagacagcacctctgttccagaagcgggcttagaccaagaacgcctcccctcatcccacctgctaactccaccatctgctgccgccaggaagcccgagccgctcggcacgaagaggagaaattctggcaaagttaactccatgtcacttcctggtttggtagagcctggcatcacctttagtaaggtagcccatgcccccgctcctcttggcctcgatgcaaaacggcggcgtctcctctaaggcccacctatcaaaaccttctgagaaatgactcggactcttcgtgcaacccggaggcacagcctccttcatcccttcccaattc

SEQ ID NO: 19014 - RNA, 3047 nt, Homo sapiens
  source 1..3047: mol_type = other RNA
tggagtccaggaatctgcattttacatatgcttctaggggatccttatgcccattaaagtttgcaaacctttatccgcccctctcaaaagtataccatcagtctaggggaagacagtcacatatgcggccaggaagaaagcaacagccctgttttggagaatgcttgcttctcccagacatatatgcatggggatgaggacccagagagtctctattgacttcaaggaaattaaccagtaactcaagcttggcttgtggctctgtaatggagagacggaggacaggtgaagaggctgtctctgaaatgagcatccccatctttccagggggcactggtatgcaggaaaaaaataacacataaaatggccagattttctacctatccttttttaagtggtgcaatcaccttttgtaagagtaaggggaacttttcttccttaatgggctaaagcatcatcaccctctcctatcctccatattcttccccttctcttaacttcctaattcctttggtggaggaggtggacaaacaagtagtcctcacaggaccaaaaccaagtttcgttttcagagtagatccaatttgaacatatcaagcacatcttccctagaagggcacagatgactggaaggcagatgtacatttctgaaaacacaaatgtcagaaccttccacccagggttggcccagcctgccatgtgaaggcaacacgagtgctatcacagatgcggcatcaggagtgtcagggtgagatcaggcatgcacatgaggtggaggaagacgagatttagagatgtccagcctttcgctggatttgagaattaacagcagactctctgtcttgccttagctctgaaggatacagcatcctttggtcactgtcagaggaagctcagttaccatcctcaaggatggtagaaaggctttccaaatccccctgggctaatccaggcagaggctggattctatcccgtccacctggaataatgcttccatcccccaaccctcatcatttgaaatttccaagaccaagataacgcatcctttcccagagacaaaggctttttgagatcatcatccatagagttctcagttagaaacaaaatgagacttgaaaggcaagttttaggattcagggttgaaccactgtcagcctggaggggacagttataaatagagggaggcgagtctcattccttcttggtgtgctctaggactcggtaggggaccccagaggcacttctggagccgtgctcttcttgcatgactggcagggtggcaggagcgtagatctcagaaatgttgtcattgttttccagagccccataggaaaaagaagctttaagttcaggctggacagtcatccctttatcgtgcatgttctgcatacctggcatggcatccatggaaatatagggctcaaatggaatgggcttcttcctgttacgcgtgattaagaagacgcccaagaatgcaatgaggcaccccagtgcaaacatgcagatgtgcagcacgtcctccccgatgaagtccaggtaaaatattgcacctgctgtgatagcaatggttgtggacagaatgtagcccacactggcaatcaaagaggagtcgtacatctgtgaggcttgactcaaaaacgcagcctgatagacggcggttgccaccatgcacacgaacatcacgtagaagatggggtagtcaagctgcaggttcccttgaatggacaagacaagcatcccagccacggccttgactgtcaccactgtcatggagccaagtaacgccaccaagagaagaatcacgacaatgttgttggcgttcttctccttgtagaagtagagcagcaagcagaacagaatgatctccaccagcatgtacaaaaggaaaggccagctcacgaggtgcctggtgacattctcgcctgtcatcttctcgtgactgttgggtgcgaatgtcaccagcaggtaggtacccacgacagccaaaccgcagccaacaaaggacaagacgtagcgcctcagaaagtctttcggtttccacttttccttgatgaatatgattcctatgatggcactagctatcacagaaactgcgctgaggggcacgatgagtgacagcggcgcgaaggcgtaggaggcgaacacacccagctcgcccagaagcatcaggaacaggcccagccaccatgtcttggtcttgaaataggcccggggatccttggagcctgccaggcggatgtggcagtacttctggaggttaagtgcaatgctgaccacgaggtgcccgaagatcgccaagagggcgccaatcaggttttccttgtaggagaaggaggcctcgcttacggcgctggagctacttgtgggaggcagctgctgcagcttcagggctgcgctgtgggatccgtccatggtggtctagtggcgcatcccacagggcctggcctaggaggtggagctgctgctaggcggggcccaggccagatgccatctctccttgtggtgttcacctccctccagcagccgtcacttcctcatgacaaaagaatacttcaaggctgttttggcagatttacagccttctcctcagcttcactcagagaagtgccaatttccgtggctctcccaggcagacagagaggggtgtgttttccagttcttgcggtgctaactcgaggagacagcacctctgttccagaagcgggcttagaccaagaacgcctcccctcatcccacctgctaactccaccatctgctgccgccaggaagcccgagccgctcggcacgaagaggagaaattctggcaaagttaactccatgtcacttcctggtttggtagagcctggcatcacctttagtaaggtagcccatgcccccgctcctcttggcctcgatgcaaaactggaaagaacattccaaggcaacgggacccaggttggcgaggcggcggcgtctcctctaaggcccacctatcaaaaccttctgagaaatgactcggactcttcgtgcaacccggaggcacagcctccttcatcccttcccaattc

SEQ ID NO: 19015 - RNA, 2772 nt, Homo sapiens
  source 1..2772: mol_type = other RNA
tggagtccaggaatctgcattttacatatgcttctaggggatccttatgcccattaaagtttgcaaacctttatccgcccctctcaaaagtataccatcagtctaggggaagacagtcacatatgcggccaggaagaaagcaacagccctgttttggagaatgcttgcttctcccagacatatatgcatggggatgaggacccagagagtctctattgacttcaaggaaattaaccagtaactcaagcttggcttgtggctctgtaatggagagacggaggacaggtgaagaggctgtctctgaaatgagcatccccatctttccagggggcactggtatgcaggaaaaaaataacacataaaatggccagattttctacctatccttttttaagtggtgcaatcaccttttgtaagagtaaggggaacttttcttccttaatgggctaaagcatcatcaccctctcctatcctccatattcttccccttctcttaacttcctaattcctttggtggaggaggtggacaaacaagtagtcctcacaggaccaaaaccaagtttcgttttcagagtagatccaatttgaacatatcaagcacatcttccctagaagggcacagatgactggaaggcagatgtacatttctgaaaacacaaatgtcagaaccttccacccagggttggcccagcctgccatgtgaaggcaacacgagtgctatcacagatgcggcatcaggagtgtcagggtgagatcaggcatgcacatgaggtggaggaagacgagatttagagatgtccagcctttcgctggatttgagaattaacagcagactctctgtcttgccttagctctgaaggatacagcatcctttggtcactgtcagaggaagctcagttaccatcctcaaggatggtagaaaggctttccaaatccccctgggctaatccaggcagaggctggattctatcccgtccacctggaataatgcttccatcccccaaccctcatcatttgaaatttccaagaccaagataacgcatcctttcccagagacaaaggctttttgagatcatcatccatagagttctcagttagaaacaaaatgagacttgaaaggcaagttttaggattcagggttgaaccactgtcagcctggaggggacagttataaatagagggaggcgagtctcattccttcttggtgtgctctaggactcggtaggggaccccagaggcacttctggagccgtgctcttcttgcatgactggcagggtggcaggagcgtagatctcagaaatgttgtcattgttttccagagccccataggaaaaagaagctttaagttcaggctggacagtcatccctttatcgtgcatgttctgcatacctggcatggcatccatggaaatatagggctcaaatggaatgggcttcttcctgttacgcgtgattaagaagacgcccaagaatgcaatgaggcaccccagtgcaaacatgcagatgtgcagcacgtcctccccgatgaagtccaggtaaaatattgcacctgctgtgatagcaatggttgtggacagaatgtagcccacactggcaatcaaagaggagtcgtacatctgtgaggcttgactcaaaaacgcagcctgatagacggcggttgccaccatgcacacgaacatcacgtagaagatggggtagtcaagctgcaggttcccttgaatggacaagacaagcatcccagccacggccttgactgtcaccactgtcatggagccaagtaacgccaccaagagaagaatcacgacaatgttgttggcgttcttctccttgtagaagtagagcagcaagcagaacagaatgatctccaccagcatgtacaaaaggaaaggccagctcacgaggtgcctggtgacattctcgcctgtcatcttctcgtgactgttgggtgcgaatgtcaccagcaggtaggtacccacgacagccaaaccgcagccaacaaaggacaagacgtagcgcctcagaaagtctttcggtttccacttttccttgatgaatatgattcctatgatggcactagctatcacagaaactgcgctgaggggcacgatgagtgacagcggcgcgaaggcgtaggaggcgaacacacccagctcgcccagaagcatcaggaacaggcccagccaccatgtcttggtcttgaaataggcccggggatccttggagcctgccaggcggatgtggcagtacttctggaggttaagtgcaatgctgaccacgaggtgcccgaagatcgccaagagggcgccaatcaggttttccttgtaggagaaggaggcctcgcttacggcgctggagctacttgtgggaggcagctgctgcagcttcagggctgcgctgtgggatccgtccatggtggtctagtggcgcatcccacagggcctggcctaggaggtggagctgctgctaggcggggcccaggccagatgccatctctccttgtggtgttcacctccctccagcagccgtcacttcctcatgacaaaagaatacttcaaggctgttttggcagatttacagccttctcctcagcttcactcagagaagtgccaatttccgtggctctcccaggcagacagagaggggtgtgttttccagttcttgcggtgctcggcggcgtctcctctaaggcccacctatcaaaaccttctgagaaatgactcggactcttcgtgcaacccggaggcacagcctccttcatcccttcccaattc

SEQ ID NO: 19016 - RNA, 2920 nt, Homo sapiens
  source 1..2920: mol_type = other RNA
tggagtccaggaatctgcattttacatatgcttctaggggatccttatgcccattaaagtttgcaaacctttatccgcccctctcaaaagtataccatcagtctaggggaagacagtcacatatgcggccaggaagaaagcaacagccctgttttggagaatgcttgcttctcccagacatatatgcatggggatgaggacccagagagtctctattgacttcaaggaaattaaccagtaactcaagcttggcttgtggctctgtaatggagagacggaggacaggtgaagaggctgtctctgaaatgagcatccccatctttccagggggcactggtatgcaggaaaaaaataacacataaaatggccagattttctacctatccttttttaagtggtgcaatcaccttttgtaagagtaaggggaacttttcttccttaatgggctaaagcatcatcaccctctcctatcctccatattcttccccttctcttaacttcctaattcctttggtggaggaggtggacaaacaagtagtcctcacaggaccaaaaccaagtttcgttttcagagtagatccaatttgaacatatcaagcacatcttccctagaagggcacagatgactggaaggcagatgtacatttctgaaaacacaaatgtcagaaccttccacccagggttggcccagcctgccatgtgaaggcaacacgagtgctatcacagatgcggcatcaggagtgtcagggtgagatcaggcatgcacatgaggtggaggaagacgagatttagagatgtccagcctttcgctggatttgagaattaacagcagactctctgtcttgccttagctctgaaggatacagcatcctttggtcactgtcagaggaagctcagttaccatcctcaaggatggtagaaaggctttccaaatccccctgggctaatccaggcagaggctggattctatcccgtccacctggaataatgcttccatcccccaaccctcatcatttgaaatttccaagaccaagataacgcatcctttcccagagacaaaggctttttgagatcatcatccatagagttctcagttagaaacaaaatgagacttgaaaggcaagttttaggattcagggttgaaccactgtcagcctggaggggacagttataaatagagggaggcgagtctcattccttcttggtgtgctctaggactcggtaggggaccccagaggcacttctggagccgtgctcttcttgcatgactggcagggtggcaggagcgtagatctcagaaatgttgtcattgttttccagagccccataggaaaaagaagctttaagttcaggctggacagtcatccctttatcgtgcatgttctgcatacctggcatggcatccatggaaatatagggctcaaatggaatgggcttcttcctgttacgcgtgattaagaagacgcccaagaatgcaatgaggcaccccagtgcaaacatgcagatgtgcagcacgtcctccccgatgaagtccaggtaaaatattgcacctgctgtgatagcaatggttgtggacagaatgtagcccacactggcaatcaaagaggagtcgtacatctgtgaggcttgactcaaaaacgcagcctgatagacggcggttgccaccatgcacacgaacatcacgtagaagatggggtagtcaagctgcaggttcccttgaatggacaagacaagcatcccagccacggccttgactgtcaccactgtcatggagccaagtaacgccaccaagagaagaatcacgacaatgttgttggcgttcttctccttgtagaagtagagcagcaagcagaacagaatgatctccaccagcatgtacaaaaggaaaggccagctcacgaggtgcctggtgacattctcgcctgtcatcttctcgtgactgttgggtgcgaatgtcaccagcaggtaggtacccacgacagccaaaccgcagccaacaaaggacaagacgtagcgcctcagaaagtctttcggtttccacttttccttgatgaatatgattcctatgatggcactagctatcacagaaactgcgctgaggggcacgatgagtgacagcggcgcgaaggcgtaggaggcgaacacacccagctcgcccagaagcatcaggaacaggcccagccaccatgtcttggtcttgaaataggcccggggatccttggagcctgccaggcggatgtggcagtacttctggaggttaagtgcaatgctgaccacgaggtgcccgaagatcgccaagagggcgccaatcaggttttccttgtaggagaaggaggcctcgcttacggcgctggagctacttgtgggaggcagctgctgcagcttcagggctgcgctgtgggatccgtccatggtggtctagtggcgcatcccacagggcctggcctaggaggtggagctgctgctaggcggggcccaggccagatgccatctctccttgtggtgttcacctccctccagcagccgtcacttcctcatgacaaaagaatacttcaaggctgttttggcagatttacagccttctcctcagcttcactcagagaagtgccaatttccgtggctctcccaggcagacagagaggggtgtgttttccagttcttgcggtgctctcgcggacggcggaaggtggactcgcgaatgttaggcctgtgggtgccatagcgaccgggaggttgggctggccagattcagctgccgggaccggaccaggtaggaagcagttccggcggggggaccggtccctgaggtcgtggggaagaggacacggcgcaccatgtcctccgcatgggacgcccgcggagaccccccggcctccgggtgcttgcggaattccagggctgagctaggtggagccccgag

SEQ ID NO: 19017 - RNA, 2877 nt, Homo sapiens
  source 1..2877: mol_type = other RNA
tggagtccaggaatctgcattttacatatgcttctaggggatccttatgcccattaaagtttgcaaacctttatccgcccctctcaaaagtataccatcagtctaggggaagacagtcacatatgcggccaggaagaaagcaacagccctgttttggagaatgcttgcttctcccagacatatatgcatggggatgaggacccagagagtctctattgacttcaaggaaattaaccagtaactcaagcttggcttgtggctctgtaatggagagacggaggacaggtgaagaggctgtctctgaaatgagcatccccatctttccagggggcactggtatgcaggaaaaaaataacacataaaatggccagattttctacctatccttttttaagtggtgcaatcaccttttgtaagagtaaggggaacttttcttccttaatgggctaaagcatcatcaccctctcctatcctccatattcttccccttctcttaacttcctaattcctttggtggaggaggtggacaaacaagtagtcctcacaggaccaaaaccaagtttcgttttcagagtagatccaatttgaacatatcaagcacatcttccctagaagggcacagatgactggaaggcagatgtacatttctgaaaacacaaatgtcagaaccttccacccagggttggcccagcctgccatgtgaaggcaacacgagtgctatcacagatgcggcatcaggagtgtcagggtgagatcaggcatgcacatgaggtggaggaagacgagatttagagatgtccagcctttcgctggatttgagaattaacagcagactctctgtcttgccttagctctgaaggatacagcatcctttggtcactgtcagaggaagctcagttaccatcctcaaggatggtagaaaggctttccaaatccccctgggctaatccaggcagaggctggattctatcccgtccacctggaataatgcttccatcccccaaccctcatcatttgaaatttccaagaccaagataacgcatcctttcccagagacaaaggctttttgagatcatcatccatagagttctcagttagaaacaaaatgagacttgaaaggcaagttttaggattcagggttgaaccactgtcagcctggaggggacagttataaatagagggaggcgagtctcattccttcttggtgtgctctaggactcggtaggggaccccagaggcacttctggagccgtgctcttcttgcatgactggcagggtggcaggagcgtagatctcagaaatgttgtcattgttttccagagccccataggaaaaagaagctttaagttcaggctggacagtcatccctttatcgtgcatgttctgcatacctggcatggcatccatggaaatatagggctcaaatggaatgggcttcttcctgttacgcgtgattaagaagacgcccaagaatgcaatgaggcaccccagtgcaaacatgcagatgtgcagcacgtcctccccgatgaagtccaggtaaaatattgcacctgctgtgatagcaatggttgtggacagaatgtagcccacactggcaatcaaagaggagtcgtacatctgtgaggcttgactcaaaaacgcagcctgatagacggcggttgccaccatgcacacgaacatcacgtagaagatggggtagtcaagctgcaggttcccttgaatggacaagacaagcatcccagccacggccttgactgtcaccactgtcatggagccaagtaacgccaccaagagaagaatcacgacaatgttgttggcgttcttctccttgtagaagtagagcagcaagcagaacagaatgatctccaccagcatgtacaaaaggaaaggccagctcacgaggtgcctggtgacattctcgcctgtcatcttctcgtgactgttgggtgcgaatgtcaccagcaggtaggtacccacgacagccaaaccgcagccaacaaaggacaagacgtagcgcctcagaaagtctttcggtttccacttttccttgatgaatatgattcctatgatggcactagctatcacagaaactgcgctgaggggcacgatgagtgacagcggcgcgaaggcgtaggaggcgaacacacccagctcgcccagaagcatcaggaacaggcccagccaccatgtcttggtcttgaaataggcccggggatccttggagcctgccaggcggatgtggcagtacttctggaggttaagtgcaatgctgaccacgaggtgcccgaagatcgccaagagggcgccaatcaggttttccttgtaggagaaggaggcctcgcttacggcgctggagctacttgtgggaggcagctgctgcagcttcagggctgcgctgtgggatccgtccatggtggtctagtggcgcatcccacagggcctggcctaggaggtggagctgctgctaggcggggcccaggccagatgccatctctccttgtggtgttcacctccctccagcagccgtcacttcctcatgacaaaagaatacttcaaggctgttttggcagatttacagccttctcctcagcttcactcagagaagtgccaatttccgtggctctcccaggcagacagagaggggtgtgttttccagttcttgcggtgctctgctaactccaccatctgctgccgccaggaagcccgagccgctcggcacgaagaggagaaattctggcaaagttaactccatgtcacttcctggtttggtagagcctggcatcacctttagtaaggtagcccatgcccccgctcctcttggcctcgatgcaaaactggaaagaacattccaaggcaacgggacccaggttggcgagg

SEQ ID NO: 19018 - RNA, 2745 nt, Homo sapiens
  source 1..2745: mol_type = other RNA
tggagtccaggaatctgcattttacatatgcttctaggggatccttatgcccattaaagtttgcaaacctttatccgcccctctcaaaagtataccatcagtctaggggaagacagtcacatatgcggccaggaagaaagcaacagccctgttttggagaatgcttgcttctcccagacatatatgcatggggatgaggacccagagagtctctattgacttcaaggaaattaaccagtaactcaagcttggcttgtggctctgtaatggagagacggaggacaggtgaagaggctgtctctgaaatgagcatccccatctttccagggggcactggtatgcaggaaaaaaataacacataaaatggccagattttctacctatccttttttaagtggtgcaatcaccttttgtaagagtaaggggaacttttcttccttaatgggctaaagcatcatcaccctctcctatcctccatattcttccccttctcttaacttcctaattcctttggtggaggaggtggacaaacaagtagtcctcacaggaccaaaaccaagtttcgttttcagagtagatccaatttgaacatatcaagcacatcttccctagaagggcacagatgactggaaggcagatgtacatttctgaaaacacaaatgtcagaaccttccacccagggttggcccagcctgccatgtgaaggcaacacgagtgctatcacagatgcggcatcaggagtgtcagggtgagatcaggcatgcacatgaggtggaggaagacgagatttagagatgtccagcctttcgctggatttgagaattaacagcagactctctgtcttgccttagctctgaaggatacagcatcctttggtcactgtcagaggaagctcagttaccatcctcaaggatggtagaaaggctttccaaatccccctgggctaatccaggcagaggctggattctatcccgtccacctggaataatgcttccatcccccaaccctcatcatttgaaatttccaagaccaagataacgcatcctttcccagagacaaaggctttttgagatcatcatccatagagttctcagttagaaacaaaatgagacttgaaaggcaagttttaggattcagggttgaaccactgtcagcctggaggggacagttataaatagagggaggcgagtctcattccttcttggtgtgctctaggactcggtaggggaccccagaggcacttctggagccgtgctcttcttgcatgactggcagggtggcaggagcgtagatctcagaaatgttgtcattgttttccagagccccataggaaaaagaagctttaagttcaggctggacagtcatccctttatcgtgcatgttctgcatacctggcatggcatccatggaaatatagggctcaaatggaatgggcttcttcctgttacgcgtgattaagaagacgcccaagaatgcaatgaggcaccccagtgcaaacatgcagatgtgcagcacgtcctccccgatgaagtccaggtaaaatattgcacctgctgtgatagcaatggttgtggacagaatgtagcccacactggcaatcaaagaggagtcgtacatctgtgaggcttgactcaaaaacgcagcctgatagacggcggttgccaccatgcacacgaacatcacgtagaagatggggtagtcaagctgcaggttcccttgaatggacaagacaagcatcccagccacggccttgactgtcaccactgtcatggagccaagtaacgccaccaagagaagaatcacgacaatgttgttggcgttcttctccttgtagaagtagagcagcaagcagaacagaatgatctccaccagcatgtacaaaaggaaaggccagctcacgaggtgcctggtgacattctcgcctgtcatcttctcgtgactgttgggtgcgaatgtcaccagcaggtaggtacccacgacagccaaaccgcagccaacaaaggacaagacgtagcgcctcagaaagtctttcggtttccacttttccttgatgaatatgattcctatgatggcactagctatcacagaaactgcgctgaggggcacgatgagtgacagcggcgcgaaggcgtaggaggcgaacacacccagctcgcccagaagcatcaggaacaggcccagccaccatgtcttggtcttgaaataggcccggggatccttggagcctgccaggcggatgtggcagtacttctggaggttaagtgcaatgctgaccacgaggtgcccgaagatcgccaagagggcgccaatcaggttttcggcgctggagctacttgtgggaggcagctgctgcagcttcagggctgcgctgtgggatccgtccatggtggtctagtggcgcatcccacagggcctggcctaggaggtggagctgctgctaggcggggcccaggccagatgccatctctccttgtggtgttcacctccctccagcagccgtcacttcctcatgacaaaagaatacttcaaggctgttttggcagatttacagccttctcctcagcttcactcagagaagtgccaatttccgtggctctcccaggcagacagagaggggtgtgttttccagttcttgcggtgctcggcggcgtctcctctaaggcccacctatcaaaaccttctgagaaatgactcggactcttcgtgcaacccggaggcacagcctccttcatcccttcccaattc

SEQ ID NO: 19019 - RNA, 2922 nt, Homo sapiens
  source 1..2922: mol_type = other RNA
tggagtccaggaatctgcattttacatatgcttctaggggatccttatgcccattaaagtttgcaaacctttatccgcccctctcaaaagtataccatcagtctaggggaagacagtcacatatgcggccaggaagaaagcaacagccctgttttggagaatgcttgcttctcccagacatatatgcatggggatgaggacccagagagtctctattgacttcaaggaaattaaccagtaactcaagcttggcttgtggctctgtaatggagagacggaggacaggtgaagaggctgtctctgaaatgagcatccccatctttccagggggcactggtatgcaggaaaaaaataacacataaaatggccagattttctacctatccttttttaagtggtgcaatcaccttttgtaagagtaaggggaacttttcttccttaatgggctaaagcatcatcaccctctcctatcctccatattcttccccttctcttaacttcctaattcctttggtggaggaggtggacaaacaagtagtcctcacaggaccaaaaccaagtttcgttttcagagtagatccaatttgaacatatcaagcacatcttccctagaagggcacagatgactggaaggcagatgtacatttctgaaaacacaaatgtcagaaccttccacccagggttggcccagcctgccatgtgaaggcaacacgagtgctatcacagatgcggcatcaggagtgtcagggtgagatcaggcatgcacatgaggtggaggaagacgagatttagagatgtccagcctttcgctggatttgagaattaacagcagactctctgtcttgccttagctctgaaggatacagcatcctttggtcactgtcagaggaagctcagttaccatcctcaaggatggtagaaaggctttccaaatccccctgggctaatccaggcagaggctggattctatcccgtccacctggaataatgcttccatcccccaaccctcatcatttgaaatttccaagaccaagataacgcatcctttcccagagacaaaggctttttgagatcatcatccatagagttctcagttagaaacaaaatgagacttgaaaggcaagttttaggattcagggttgaaccactgtcagcctggaggggacagttataaatagagggaggcgagtctcattccttcttggtgtgctctaggactcggtaggggaccccagaggcacttctggagccgtgctcttcttgcatgactggcagggtggcaggagcgtagatctcagaaatgttgtcattgttttccagagccccataggaaaaagaagctttaagttcaggctggacagtcatccctttatcgtgcatgttctgcatacctggcatggcatccatggaaatatagggctcaaatggaatgggcttcttcctgttacgcgtgattaagaagacgcccaagaatgcaatgaggcaccccagtgcaaacatgcagatgtgcagcacgtcctccccgatgaagtccaggtaaaatattgcacctgctgtgatagcaatggttgtggacagaatgtagcccacactggcaatcaaagaggagtcgtacatctgtgaggcttgactcaaaaacgcagcctgatagacggcggttgccaccatgcacacgaacatcacgtagaagatggggtagtcaagctgcaggttcccttgaatggacaagacaagcatcccagccacggccttgactgtcaccactgtcatggagccaagtaacgccaccaagagaagaatcacgacaatgttgttggcgttcttctccttgtagaagtagagcagcaagcagaacagaatgatctccaccagcatgtacaaaaggaaaggccagctcacgaggtgcctggtgacattctcgcctgtcatcttctcgtgactgttgggtgcgaatgtcaccagcaggtaggtacccacgacagccaaaccgcagccaacaaaggacaagacgtagcgcctcagaaagtctttcggtttccacttttccttgatgaatatgattcctatgatggcactagctggagcagtgatggttaagtcatagatatccaataagtgataatcattattatttttaatattactcctcactggatgacctcagaagctatagggccccttcatttccagtggctgatatctgaagttttatcattataacttggcctctatcacagaaactgcgctgaggggcacgatgagtgacagcggcgcgaaggcgtaggaggcgaacacacccagctcgcccagaagcatcaggaacaggcccagccaccatgtcttggtcttgaaataggcccggggatccttggagcctgccaggcggatgtggcagtacttctggaggttaagtgcaatgctgaccacgaggtgcccgaagatcgccaagagggcgccaatcaggttttccttgtaggagaaggaggcctcgcttacggcgctggagctacttgtgggaggcagctgctgcagcttcagggctgcgctgtgggatccgtccatggtggtctagtggcgcatcccacagggcctggcctaggaggtggagctgctgctaggcggggcccaggccagatgccatctctccttgtggtgttcacctccctccagcagccgtcacttcctcatgacaaaagaatacttcaaggctgttttggcagatttacagccttctcctcagcttcactcagagaagtgccaatttccgtggctctcccaggcagacagagaggggtgtgttttccagttcttgcggtgctcggcggcgtctcctctaaggcccacctatcaaaaccttctgagaaatgactcggactcttcgtgcaacccggaggcacagcctccttcatcccttcccaattc

SEQ ID NO: 19020 - RNA, 2531 nt, Homo sapiens
  source 1..2531: mol_type = other RNA
tggagtccaggaatctgcattttacatatgcttctaggggatccttatgcccattaaagtttgcaaacctttatccgcccctctcaaaagtataccatcagtctaggggaagacagtcacatatgcggccaggaagaaagcaacagccctgttttggagaatgcttgcttctcccagacatatatgcatggggatgaggacccagagagtctctattgacttcaaggaaattaaccagtaactcaagcttggcttgtggctctgtaatggagagacggaggacaggtgaagaggctgtctctgaaatgagcatccccatctttccagggggcactggtatgcaggaaaaaaataacacataaaatggccagattttctacctatccttttttaagtggtgcaatcaccttttgtaagagtaaggggaacttttcttccttaatgggctaaagcatcatcaccctctcctatcctccatattcttccccttctcttaacttcctaattcctttggtggaggaggtggacaaacaagtagtcctcacaggaccaaaaccaagtttcgttttcagagtagatccaatttgaacatatcaagcacatcttccctagaagggcacagatgactggaaggcagatgtacatttctgaaaacacaaatgtcagaaccttccacccagggttggcccagcctgccatgtgaaggcaacacgagtgctatcacagatgcggcatcaggagtgtcagggtgagatcaggcatgcacatgaggtggaggaagacgagatttagagatgtccagcctttcgctggatttgagaattaacagcagactctctgtcttgccttagctctgaaggatacagcatcctttggtcactgtcagaggaagctcagttaccatcctcaaggatggtagaaaggctttccaaatccccctgggctaatccaggcagaggctggattctatcccgtccacctggaataatgcttccatcccccaaccctcatcatttgaaatttccaagaccaagataacgcatcctttcccagagacaaaggctttttgagatcatcatccatagagttctcagttagaaacaaaatgagacttgaaaggcaagttttaggattcagggttgaaccactgtcagcctggaggggacagttataaatagagggaggcgagtctcattccttcttggtgtgctctaggactcggtaggggaccccagaggcacttctggagccgtgctcttcttgcatgactggcagggtggcaggagcgtagatctcagaaatgttgtcattgttttccagagccccataggaaaaagaagctttaagttcaggctggacagtcatccctttatcgtgcatgttctgcatacctggcatggcatccatggaaatatagggctcaaatggaatgggcttcttcctgttacgcgtgattaagaagacgcccaagaatgcaatgaggcaccccagtgcaaacatgcagatgtgcagcacgtcctccccgatgaagtccaggtaaaatattgcacctgctgtgatagcaatggttgtggacagaatgtagcccacactggcaatcaaagaggagtcgtacatctgtgaggcttgactcaaaaacgcagcctgatagacggcggttgccaccatgcacacgaacatcacgtagaagatggggtagtcaagctgcaggttcccttgaatggacaagacaagcatcccagccacggccttgactgtcaccactgtcatggagccaagtaacgccaccaagagaagaatcacgacaatgttgttggcgttcttctccttgtagaagtagagcagcaagcagaacagaatgatctccaccagcatgtacaaaaggaaaggccagctcacgaggtgcctggtgacattctcgcctgtcatcttctcgtgactgttgggtgcgaatgtcaccagcaggtaggtacccacgacagccaaaccgcagccaacaaaggacaagacgtagcgcctcagaaagtctttcggtttccacttttccttgatgaatatgattcctatgatggcactagcttgtaggagaaggaggcctcgcttacggcgctggagctacttgtgggaggcagctgctgcagcttcagggctgcgctgtgggatccgtccatggtggtctagtggcgcatcccacagggcctggcctaggaggtggagctgctgctaggcggggcccaggccagatgccatctctccttgtggtgttcacctccctccagcagccgtcacttcctcatgacaaaagaatacttcaaggctgttttggcagatttacagccttctcctcagcttcactcagagaagtgccaatttccgtggctctcccaggcagacagagaggggtgtgttttccagttcttgcggtgctcggcggcgtctcctctaaggcccacctatcaaaaccttctgagaaatgactcggactcttcgtgcaacccggaggcacagcctccttcatcccttcccaattc

SEQ ID NO: 19021 - RNA, 2675 nt, Homo sapiens
  source 1..2675: mol_type = other RNA
tggagtccaggaatctgcattttacatatgcttctaggggatccttatgcccattaaagtttgcaaacctttatccgcccctctcaaaagtataccatcagtctaggggaagacagtcacatatgcggccaggaagaaagcaacagccctgttttggagaatgcttgcttctcccagacatatatgcatggggatgaggacccagagagtctctattgacttcaaggaaattaaccagtaactcaagcttggcttgtggctctgtaatggagagacggaggacaggtgaagaggctgtctctgaaatgagcatccccatctttccagggggcactggtatgcaggaaaaaaataacacataaaatggccagattttctacctatccttttttaagtggtgcaatcaccttttgtaagagtaaggggaacttttcttccttaatgggctaaagcatcatcaccctctcctatcctccatattcttccccttctcttaacttcctaattcctttggtggaggaggtggacaaacaagtagtcctcacaggaccaaaaccaagtttcgttttcagagtagatccaatttgaacatatcaagcacatcttccctagaagggcacagatgactggaaggcagatgtacatttctgaaaacacaaatgtcagaaccttccacccagggttggcccagcctgccatgtgaaggcaacacgagtgctatcacagatgcggcatcaggagtgtcagggtgagatcaggcatgcacatgaggtggaggaagacgagatttagagatgtccagcctttcgctggatttgagaattaacagcagactctctgtcttgccttagctctgaaggatacagcatcctttggtcactgtcagaggaagctcagttaccatcctcaaggatggtagaaaggctttccaaatccccctgggctaatccaggcagaggctggattctatcccgtccacctggaataatgcttccatcccccaaccctcatcatttgaaatttccaagaccaagataacgcatcctttcccagagacaaaggctttttgagatcatcatccatagagttctcagttagaaacaaaatgagacttgaaaggcaagttttaggattcagggttgaaccactgtcagcctggaggggacagttataaatagagggaggcgagtctcattccttcttggtgtgctctaggactcggtaggggaccccagaggcacttctggagccgtgctcttcttgcatgactggcagggtggcaggagcgtagatctcagaaatgttgtcattgttttccagagccccataggaaaaagaagctttaagttcaggctggacagtcatccctttatcgtgcatgttctgcatacctggcatggcatccatggaaatatagggctcaaatggaatgggcttcttcctgttacgcgtgattaagaagacgcccaagaatgcaatgaggcaccccagtgcaaacatgcagatgtgcagcacgtcctccccgatgaagtccaggtaaaatattgcacctgctgtgatagcaatggttgtggacagaatgtagcccacactggcaatcaaagaggagtcgtacatctgtgaggcttgactcaaaaacgcagcctgatagacggcggttgccaccatgcacacgaacatcacgtagaagatggggtagtcaagctgcaggttcccttgaatggacaagacaagcatcccagccacggccttgactgtcaccactgtcatggagccatgtacaaaaggaaaggccagctcacgaggtgcctggtgacattctcgcctgtcatcttctcgtgactgttgggtgcgaatgtcaccagcaggtaggtacccacgacagccaaaccgcagccaacaaaggacaagacgtagcgcctcagaaagtctttcggtttccacttttccttgatgaatatgattcctatgatggcactagctatcacagaaactgcgctgaggggcacgatgagtgacagcggcgcgaaggcgtaggaggcgaacacacccagctcgcccagaagcatcaggaacaggcccagccaccatgtcttggtcttgaaataggcccggggatccttggagcctgccaggcggatgtggcagtacttctggaggttaagtgcaatgctgaccacgaggtgcccgaagatcgccaagagggcgccaatcaggttttccttgtaggagaaggaggcctcgcttacggcgctggagctacttgtgggaggcagctgctgcagcttcagggctgcgctgtgggatccgtccatggtggtctagtggcgcatcccacagggcctggcctaggaggtggagctgctgctaggcggggcccaggccagatgccatctctccttgtggtgttcacctccctccagcagccgtcacttcctcatgacaaaagaatacttcaaggctgttttggcagatttacagccttctcctcagcttcactcagagaagtgccaatttccgtggctctcccaggcagacagagaggggtgtgttttccagttcttgcggtgctcggcggcgtctcctctaaggcccacctatcaaaaccttctgagaaatgactcggactcttcgtgcaacccggaggcacagcctccttcatcccttcccaattc

SEQ ID NO: 19022 - RNA, 2619 nt, Homo sapiens
  source 1..2619: mol_type = other RNA
tggagtccaggaatctgcattttacatatgcttctaggggatccttatgcccattaaagtttgcaaacctttatccgcccctctcaaaagtataccatcagtctaggggaagacagtcacatatgcggccaggaagaaagcaacagccctgttttggagaatgcttgcttctcccagacatatatgcatggggatgaggacccagagagtctctattgacttcaaggaaattaaccagtaactcaagcttggcttgtggctctgtaatggagagacggaggacaggtgaagaggctgtctctgaaatgagcatccccatctttccagggggcactggtatgcaggaaaaaaataacacataaaatggccagattttctacctatccttttttaagtggtgcaatcaccttttgtaagagtaaggggaacttttcttccttaatgggctaaagcatcatcaccctctcctatcctccatattcttccccttctcttaacttcctaattcctttggtggaggaggtggacaaacaagtagtcctcacaggaccaaaaccaagtttcgttttcagagtagatccaatttgaacatatcaagcacatcttccctagaagggcacagatgactggaaggcagatgtacatttctgaaaacacaaatgtcagaaccttccacccagggttggcccagcctgccatgtgaaggcaacacgagtgctatcacagatgcggcatcaggagtgtcagggtgagatcaggcatgcacatgaggtggaggaagacgagatttagagatgtccagcctttcgctggatttgagaattaacagcagactctctgtcttgccttagctctgaaggatacagcatcctttggtcactgtcagaggaagctcagttaccatcctcaaggatggtagaaaggctttccaaatccccctgggctaatccaggcagaggctggattctatcccgtccacctggaataatgcttccatcccccaaccctcatcatttgaaatttccaagaccaagataacgcatcctttcccagagacaaaggctttttgagatcatcatccatagagttctcagttagaaacaaaatgagacttgaaaggcaagttttaggattcagggttgaaccactgtcagcctggaggggacagttataaatagagggaggcgagtctcattccttcttggtgtgctctaggactcggtaggggaccccagaggcacttctggagccgtgctcttcttgcatgactggcagggtggcaggagcgtagatctcagaaatgttgtcattgttttccagagccccataggaaaaagaagctttaagttcaggctggacagtcatccctttatcgtgcatgttctgcatacctggcatggcatccatggaaatatagggctcaaatggaatgggcttcttcctgttacgcgtgattaagaagacgcccaagaatgcaatgaggcacgcagcctgatagacggcggttgccaccatgcacacgaacatcacgtagaagatggggtagtcaagctgcaggttcccttgaatggacaagacaagcatcccagccacggccttgactgtcaccactgtcatggagccaagtaacgccaccaagagaagaatcacgacaatgttgttggcgttcttctccttgtagaagtagagcagcaagcagaacagaatgatctccaccagcatgtacaaaaggaaaggccagctcacgaggtgcctggtgacattctcgcctgtcatcttctcgtgactgttgggtgcgaatgtcaccagcaggtaggtacccacgacagccaaaccgcagccaacaaaggacaagacgtagcgcctcagaaagtctttcggtttccacttttccttgatgaatatgattcctatgatggcactagctatcacagaaactgcgctgaggggcacgatgagtgacagcggcgcgaaggcgtaggaggcgaacacacccagctcgcccagaagcatcaggaacaggcccagccaccatgtcttggtcttgaaataggcccggggatccttggagcctgccaggcggatgtggcagtacttctggaggttaagtgcaatgctgaccacgaggtgcccgaagatcgccaagagggcgccaatcaggttttccttgtaggagaaggaggcctcgcttacggcgctggagctacttgtgggaggcagctgctgcagcttcagggctgcgctgtgggatccgtccatggtggtctagtggcgcatcccacagggcctggcctaggaggtggagctgctgctaggcggggcccaggccagatgccatctctccttgtggtgttcacctccctccagcagccgtcacttcctcatgacaaaagaatacttcaaggctgttttggcagatttacagccttctcctcagcttcactcagagaagtgccaatttccgtggctctcccaggcagacagagaggggtgtgttttccagttcttgcggtgctcggcggcgtctcctctaaggcccacctatcaaaaccttctgagaaatgactcggactcttcgtgcaacccggaggcacagcctccttcatcccttcccaattc

SEQ ID NO: 19023 - RNA, 1425 nt, Homo sapiens
  source 1..1425: mol_type = other RNA
tggagtccaggaatctgcattttcaacgatcttctaggtgcttcttataaagattaggaaccactgagcccaactgtcaataattgtaactttttgcctgtttgccatataaccctttgagaaccactgtctctatccattcctggtgttctagagttgtttcattactacctgcaacagcagcttattcaatctttagtagtcacaagcattcaccaagcaatctaggtaagtttatctctataggaggaaaacacctttcctttaaatacgtcacaaattatatatatttattaaaatatgagagcaaagaattaaaccttgagaattaggatgaaccaggcctttcttttttaatagaatctcgttaaatcctggcatttacttcaaatagaaataatacaaagaaaccaaagagaacaaaatctgagtctgtttttttttttgtttggttggtttttcttcttttttaaaaaaatttcaacagctttaggggtacaagcagcttttggtaacacagataaattgtaggatgatgaagtctgggcttttattgtacccttcgcccaagcggtgtacactgcacccagcagtcatttctgagtctgattaattcaggttttttttaaaagaaccagaagctccaacatacctgataattcatgatggcacgtaaacacatgatacagacatgcacatcatctttcttactcactaatcttgaatttttcagagttcttctgcttggcaatgtattatatcgcagtgcagaatgtcttccagagcgggagacactgttgcccacaggtgagggcaggttgctccctctgtgcaggtcctcgatggacctactccagggctttgatttgtccaccgagctctccacagtactctccacactttcaaagtcaaaagttaccgcgtactgtgcaaatgagagatattccactagaacatcaagacctttgttttcttcattcagaaattctctgacccatccaatgtggttagttctcaaagaaatttccagttctcttagcacttgtgtagattcttgaacacgccgtctgaatttcttcctggttacagctggatccagatagcctttgagcttttgaatgtatgtatggggaggattcttcacctggaatcgttcctgatcacaaatcagttcccattttttctcattatcatactgccgcagtaacctggctttgtcaggaggtaggttcatagcattcagcacgatggcaaatcgctcctccagttcacctggctctggcatcggcagcttcaaaggcacgttgtgcgccctgaaatcggtctgctgcgaatccatgctccctgcgttgcccatgtcggcggcgcgccggggccgggggctgctccgggcccctagcgtgcgcgtcggaaatcagaacagct

SEQ ID NO: 19024 - RNA, 3129 nt, Homo sapiens
  source 1..3129: mol_type = other RNA
tggagtccaggaatctgcattttctcctggaaggaactgaagtggagctatgccaattccaatcaaatgatctttgtgtattttttcataactttcggccaaaacagctttcacacccagtaaatacggtcctttggcagcccagtctctggagtttcctgaaccatatttctttcctgctaaaataatcagtgggataccttctttctggtacagctctgcagcctcaaatacatctagcgtctgtcctgatggaaaatgaattgttttaggagctggttttccaataaacttattaaaaagcttgatatttgcaaaagtgcctcttgtcattacagcatcattacctcttcgagctccgtaagagttgaattcacgaggggtaaggcctctgtttgtcaaatacttagcggcagcactattcctagcgatacttcctgcaggtgatatatgatctgttgtgacagagtctcccaaatataataagacatgggcattttcaatagcctggagtgcaattggctctttggtaagtttatcaaaaaatgaagggcatctgatataagtagactttaagtcccatggaaacaaaactgaatccggtgcttctaaggaattccaccgtttattccccatttctattttatcttttaatgctttaaacatggatagtataacatgttcttcctctactcgatgaacttcttctcgactaggccaaatatcatgcaggtaaatgttcttgccggtggggtcagtacctaaaggttctgtctggaaatctatattcactgtgcctgctatggcataagctaccactaagggtggagaggcaagataattggcacgaacacaatcacaaagacgaccttcaaaatttttgtttccagataaaattccacaggtaaccaaatcaccctgttttactgcatttaaaactgcgtctgataagggtgctgtatttcccacacaaattgaacatccatagccaacgatttcaaatccaagcttacttagatatggtaatactccacttgaactgaggtaatgtgtaaccatcccactgcctggagataaacttgttcttatataaggtttaacacgcagaccagcttcaacagcctttttagccaaaagacctgcagcaagcatgacagatggattgcaattattggtacaactgataactgcagcaatgaccactgatccatgagacagcttatattcacttccttcataatgaatggagacaatatccttttgtttttcagctgcaatttggaagcctttaaatccaaccttttcatttaagcaagcctggaaatcgcttttcatatctgtcacagcaactctatcctgaggtctttttggaccactaacagatggaactattgaattcagattaatctggatcacctgggagtattcaggttctcctgaagaattctggtcatttcgaaacaatttcacagctttaaggtatgtttccattgattcgagtttggctttgctaaaacctgtatgttctaaatgttttaatgtcacattgtcaacagggaaaaagctgaggatagcaccatattccggacacatgtttgctattgtagttcgatcaactatagataattgtgaaactccacttccaaaaaactcaacaaactttccagccactcctacttgcctgaggtgctttgtaataccaagaacaacatctatggatgtaacaaaagggtttgatgacccagttaactcacatccaaccacctctggtaaagtaagagaaactggcagaccaagcataactgcttctgtttcaatgcctccaaccccccaccccagaatccctaaaccattcaccatcgttatgtgtgaatctgtgccgactacactgtctgggaagaggaggtctttttcttcaaaaaccactcttgacaaatattctaagtttatttgatgagccattccagttccaggagggatcactgccacattcttaaaaactcttgaactccacttaaaaaactgaagcctctctcgatttctgccgaattctacttcttgattttttaacactgtttcaggttcaggcactggttgcaaatgaaaaggacacaggatgggtgtattctcaatctgcgaagaaaatgttcctgagtttcggcctagttctccagaatcacaagatcctcggcaggtagtctggcctctgcagggaagcttcttaggctgcactttaagtggagagagctttcctgctttctgcaggtcaccacctccaggatttggtgcattctgtattgcacatttactgaagtcaatttgtaaagaatggtcaactgtaagatctgtcggacaagcaggatggactttctcaggatcacctccaagagttttcactgcctccctcatagcagcaaaatccaccattgctggtattccagtaaaatcttgaagaagaacacgggcagggaaaaagggcacttcaacattgctttgtttggttttccagtctaaaatgttcataacatcttccttcttcattaaaaagccatcacaatttcgtacagcagcttccaacaagacccgtattgagtaaggcagaacatcatacttggtgccaagtttagatacatcgaagaacttcttatgtgaactgtcatttaatgtttcaataaggtactcaaaggcgtatccaatgttcaaccttgactgcccctcattcggcttccagaggcacagagagactgaggggccttaggctggaccgtggaatcaacatctagctgcgtgagacccgaacacggagacgcaggcccccgccttcatcgctcgccaatggggggcgggcaggagaagacggtgggcctctccctgcccctggtgttgctgacgggggccaggaagccgctggcagcaggcagcggccaccggagagagaggggtgcgggtcaaggccagcggtggggtggcccgccctgcgggtgtcgcgcaggagggtggggatcgggagccccagcttccgcggcctaggctcaaagggcggcccagcaggcaggccccgaggggagcacaacccgagccccgagggcctgggcgcctgccgagcgactccaggcgagaaaagcaagg

SEQ ID NO: 19025 - RNA, 2984 nt, Homo sapiens
  source 1..2984: mol_type = other RNA
tggagtccaggaatctgcattttctcctggaaggaactgaagtggagctatgccaattccaatcaaatgatctttgtgtattttttcataactttcggccaaaacagctttcacacccagtaaatacggtcctttggcagcccagtctctggagtttcctgaaccatatttctttcctgctaaaataatcagtgggataccttctttctggtacagctctgcagcctcaaatacatctagcgtctgtcctgatggaaaatgaattgttttaggagctggttttccaataaacttattaaaaagcttgatatttgcaaaagtgcctcttgtcattacagcatcattacctcttcgagctccgtaagagttgaattcacgaggggtaaggcctctgtttgtcaaatacttagcggcagcactattcctagcgatacttcctgcaggtgatatatgatctgttgtgacagagtctcccaaatataataagacatgggcattttcaatagcctggagtgcaattggctctttggtaagtttatcaaaaaatgaagggcatctgatataagtagactttaagtcccatggaaacaaaactgaatccggtgcttctaaggaattccaccgtttattccccatttctattttatcttttaatgctttaaacatggatagtataacatgttcttcctctactcgatgaacttcttctcgactaggccaaatatcatgcaggtaaatgttcttgccggtggggtcagtacctaaaggttctgtctggaaatctatattcactgtgcctgctatggcataagctaccactaagggtggagaggcaagataattggcacgaacacaatcacaaagacgaccttcaaaatttttgtttccagataaaattccacaggtaaccaaatcaccctgttttactgcatttaaaactgcgtctgataagggtgctgtatttcccacacaaattgaacatccatagccaacgatttcaaatccaagcttacttagatatggtaatactccacttgaactgaggtaatgtgtaaccatcccactgcctggagataaacttgttcttatataaggtttaacacgcagaccagcttcaacagcctttttagccaaaagacctgcagcaagcatgacagatggattgcaattattggtacaactgataactgcagcaatgaccactgatccatgagacagcttatattcacttccttcataatgaatggagacaatatccttttgtttttcagctgcaatttggaagcctttaaatccaaccttttcatttaagcaagcctggaaatcgcttttcatatctgtcacagcaactctatcctgaggtctttttggaccactaacagatggaactattgaattcagattaatctggatcacctgggagtattcaggttctcctgaagaattctggtcatttcgaaacaatttcacagctttaaggtatgtttccattgattcgagtttggctttgctaaaacctgtatgttctaaatgttttaatgtcacattgtcaacagggaaaaagctgaggatagcaccatattccggacacatgtttgctattgtagttcgatcaactatagataattgtgaaactccacttccaaaaaactcaacaaactttccagccactcctacttgcctgaggtgctttgtaataccaagaacaacatctatggatgtaacaaaagggtttgatgacccagttaactcacatccaaccacctctggtaaagtaagagaaactggcagaccaagcataactgcttctgtttcaatgcctccaaccccccaccccagaatccctaaaccattcaccatcgttatgtgtgaatctgtgccgactacactgtctgggaagaggaggtctttttcttcaaaaaccactcttgacaaatattctaagtttatttgatgagccattccagttccaggagggatcactgccacattcttaaaaactcttgaactccacttaaaaaactgaagcctctctcgatttctgccgaattctacttcttgattttttaacactgtttcaggttcaggcactggttgcaaatgaaaaggacacaggatgggtgtattctcaatctgcgaagaaaatgttcctgagtttcggcctagttctccagaatcacaagatcctcggcaggtagtctggcctctgcagggaagcttcttaggctgcactttaagtggagagagctttcctgctttctgcaggtcaccacctccaggatttggtgcattctgtattgcacatttactgaagtcaatttgtaaagaatggtcaactgtaagatctgtcggacaagcaggatggactttctcaggatcacctccaagagttttcactgcctccctcatagcagcaaaatccaccattgctggtattccagtaaaatcttgaagaagaacacgggcagggaaaaagggcacttcaacattgctttgtttggttttccagtctaaaatgttcataacatcttccttcttcattaaaaagccatcacaatttcgtacagcagcttccaacaagacccgtattgagtaaggcagaacatcatacttggtgccaagtttagatacatcgaagaacttcttatgtgaactgtcatttaatgtttcaataaggtactcaaaggcgtatccctccggtagcttccgtgattgccgacttcttcccagtggcagttaacacatgcttaagcctctccatccttccgcctcagctcctccggtccctgtgttctccacctacccagcattatctcctgtcgcagcaacttaccagaaagagtcgctcatactcggctctcccccacccacttcttatcctcttccagtctggcttccactcccagaaatgcctttagccaaggccagctataactccactttctaatctcacatatctcaatcttgactggttctctcccatt

SEQ ID NO: 19026 - RNA, 2834 nt, Homo sapiens
  source 1..2834: mol_type = other RNA
tggagtccaggaatctgcattttctcctggaaggaactgaagtggagctatgccaattccaatcaaatgatctttgtgtattttttcataactttcggccaaaacagctttcacacccagtaaatacggtcctttggcagcccagtctctggagtttcctgaaccatatttctttcctgctaaaataatcagtgggataccttctttctggtacagctctgcagcctcaaatacatctagcgtctgtcctgatggaaaatgaattgttttaggagctggttttccaataaacttattaaaaagcttgatatttgcaaaagtgcctcttgtcattacagcatcattacctcttcgagctccgtaagagttgaattcacgaggggtaaggcctctgtttgtcaaatacttagcggcagcactattcctagcgatacttcctgcaggtgatatatgatctgttgtgacagagtctcccaaatataataagacatgggcattttcaatagcctggagtgcaattggctctttggtaagtttatcaaaaaatgaagggcatctgatataagtagactttaagtcccatggaaacaaaactgaatccggtgcttctaaggaattccaccgtttattccccatttctattttatcttttaatgctttaaacatggatagtataacatgttcttcctctactcgatgaacttcttctcgactaggccaaatatcatgcaggtaaatgttcttgccggtggggtcagtacctaaaggttctgtctggaaatctatattcactgtgcctgctatggcataagctaccactaagggtggagaggcaagataattggcacgaacacaatcacaaagacgaccttcaaaatttttgtttccagataaaattccacaggtaaccaaatcaccctgttttactgcatttaaaactgcgtctgataagggtgctgtatttcccacacaaattgaacatccatagccaacgatttcaaatccaagcttacttagatatggtaatactccacttgaactgaggtaatgtgtaaccatcccactgcctggagataaacttgttcttatataaggtttaacacgcagaccagcttcaacagcctttttagccaaaagacctgcagcaagcatgacagatggattgcaattattggtacaactgataactgcagcaatgaccactgatccatgagacagcttatattcacttccttcataatgaatggagacaatatccttttgtttttcagctgcaatttggaagcctttaaatccaaccttttcatttaagcaagcctggaaatcgcttttcatatctgtcacagcaactctatcctgaggtctttttggaccactaacagatggaactattgaattcagattaatctggatcacctgggagtattcaggttctcctgaagaattctggtcatttcgaaacaatttcacagctttaaggtatgtttccattgattcgagtttggctttgctaaaacctgtatgttctaaatgttttaatgtcacattgtcaacagggaaaaagctgaggatagcaccatattccggacacatgtttgctattgtagttcgatcaactatagataattgtgaaactccacttccaaaaaactcaacaaactttccagccactcctacttgcctgaggtgctttgtaataccaagaacaacatctatggatgtaacaaaagggtttgatgacccagttaactcacatccaaccacctctggtaaagtaagagaaactggcagaccaagcataactgcttctgtttcaatgcctccaaccccccaccccagaatccctaaaccattcaccatcgttatgtgtgaatctgtgccgactacactgtctgggaagaggaggtctttttcttcaaaaaccactcttgacaaatattctaagtttatttgatgagccattccagttccaggagggatcactgccacattcttaaaaactcttgaactccacttaaaaaactgaagcctctctcgatttctgccgaattctacttcttgattttttaacactgtttcaggttcaggcactggttgcaaatgaaaaggacacaggatgggtgtattctcaatctgcgaagaaaatgttcctgagtttcggcctagttctccagaatcacaagatcctcggcaggtagtctggcctctgcagggaagcttcttaggctgcactttaagtggagagagctttcctgctttctgcaggtcaccacctccaggatttggtgcattctgtattgcacatttactgaagtcaatttgtaaagaatggtcaactgtaagatctgtcggacaagcaggatggactttctcaggatcacctccaagagttttcactgcctccctcatagcagcaaaatccaccattgctggtattccagtaaaatcttgaagaagaacacgggcagggaaaaagggcacttcaacattgctttgtttggttttccagtctaaaatgttcataacatcttccttcttcattaaaaagccatcacaatttcgtacagcagcttccaacaagacccgtattgagtaaggcagaacatcatacttggtgccaagtttagatacatcgaagaacttcttatgtgaactgtcatttaatgtttcaataaggtactcaaaggcgtatcctgcttttggggcgtccatcgccggagaccatattatccctccggggagggggccagcgggggaagaagggggaggccgggcagggaagacggggaggaagacaggcggactggcaagggaggaaagaaggaagcaggctc

SEQ ID NO: 19027 - RNA, 2764 nt, Homo sapiens
  source 1..2764: mol_type = other RNA
tggagtccaggaatctgcattttctcctggaaggaactgaagtggagctatgccaattccaatcaaatgatctttgtgtattttttcataactttcggccaaaacagctttcacacccagtaaatacggtcctttggcagcccagtctctggagtttcctgaaccatatttctttcctgctaaaataatcagtgggataccttctttctggtacagctctgcagcctcaaatacatctagcgtctgtcctgatggaaaatgaattgttttaggagctggttttccaataaacttattaaaaagcttgatatttgcaaaagtgcctcttgtcattacagcatcattacctcttcgagctccgtaagagttgaattcacgaggggtaaggcctctgtttgtcaaatacttagcggcagcactattcctagcgatacttcctgcaggtgatatatgatctgttgtgacagagtctcccaaatataataagacatgggcattttcaatagcctggagtgcaattggctctttggtaagtttatcaaaaaatgaagggcatctgatataagtagactttaagtcccatggaaacaaaactgaatccggtgcttctaaggaattccaccgtttattccccatttctattttatcttttaatgctttaaacatggatagtataacatgttcttcctctactcgatgaacttcttctcgactaggccaaatatcatgcaggtaaatgttcttgccggtggggtcagtacctaaaggttctgtctggaaatctatattcactgtgcctgctatggcataagctaccactaagggtggagaggcaagataattggcacgaacacaatcacaaagacgaccttcaaaatttttgtttccagataaaattccacaggtaaccaaatcaccctgttttactgcatttaaaactgcgtctgataagggtgctgtatttcccacacaaattgaacatccatagccaacgatttcaaatccaagcttacttagatatggtaatactccacttgaactgaggtaatgtgtaaccatcccactgcctggagataaacttgttcttatataaggtttaacacgcagaccagcttcaacagcctttttagccaaaagacctgcagcaagcatgacagatggattgcaattattggtacaactgataactgcagcaatgaccactgatccatgagacagcttatattcacttccttcataatgaatggagacaatatccttttgtttttcagctgcaatttggaagcctttaaatccaaccttttcatttaagcaagcctggaaatcgcttttcatatctgtcacagcaactctatcctgaggtctttttggaccactaacagatggaactattgaattcagattaatctggatcacctgggagtattcaggttctcctgaagaattctggtcatttcgaaacaatttcacagctttaaggtatgtttccattgattcgagtttggctttgctaaaacctgtatgttctaaatgttttaatgtcacattgtcaacagggaaaaagctgaggatagcaccatattccggacacatgtttgctattgtagttcgatcaactatagataattgtgaaactccacttccaaaaaactcaacaaactttccagccactcctacttgcctgaggtgctttgtaataccaagaacaacatctatggatgtaacaaaagggtttgatgacccagttaactcacatccaaccacctctggtaaagtaagagaaactggcagaccaagcataactgcttctgtttcaatgcctccaaccccccaccccagaatccctaaaccattcaccatcgttatgtgtgaatctgtgccgactacactgtctgggaagaggaggtctttttcttcaaaaaccactcttgacaaatattctaagtttatttgatgagccattccagttccaggagggatcactgccacattcttaaaaactcttgaactccatcaggcactggttgcaaatgaaaaggacacaggatgggtgtattctcaatctgcgaagaaaatgttcctgagtttcggcctagttctccagaatcacaagatcctcggcaggtagtctggcctctgcagggaagcttcttaggctgcactttaagtggagagagctttcctgctttctgcaggtcaccacctccaggatttggtgcattctgtattgcacatttactgaagtcaatttgtaaagaatggtcaactgtaagatctgtcggacaagcaggatggactttctcaggatcacctccaagagttttcactgcctccctcatagcagcaaaatccaccattgctggtattccagtaaaatcttgaagaagaacacgggcagggaaaaagggcacttcaacattgctttgtttggttttccagtctaaaatgttcataacatcttccttcttcattaaaaagccatcacaatttcgtacagcagcttccaacaagacccgtattgagtaaggcagaacatcatacttggtgccaagtttagatacatcgaagaacttcttatgtgaactgtcatttaatgtttcaataaggtactcaaaggcgtatcctgcttttggggcgtccatcgccggagaccatattatccctccggggagggggccagcgggggaagaagggggaggccgggcagggaagacggggaggaagacaggcggactggcaagggaggaaagaaggaagcaggctc

SEQ ID NO: 19028 - RNA, 2231 nt, Homo sapiens
  source 1..2231: mol_type = other RNA
tggagtccaggaatctgcattttgaacaagattcacgactattttattttattttatcacccaagctggagtgcagtggtgcaatctcggctcactgcaacctctgcctcctgagttaaagtgatactcaattcttgtgcctcagcctcctgagtaactgggattacaaacgtgcaccacacacctggttaacttttgtatttttagtagagatgaggtttcgccatgatggccaggctggtctcgaactcctgacctcaagtgattgcctgcctcagcctcccaaagtgctaggattacaggcatgaggcaccgcacccagccaagatccatgattttgatgaagtggtacaagaacctcactcactggacattgaaattctactgtccaatcccaactcactgctgttgattggaaacctgattctggcagctcatttatcttggtttcctcatttgtaaggtcgttcagttggactgatcatctctgagggccttgaagccctaacaagtctatcatgatcccagatgtaaaatatatatatgtgtatatatataatttcagctgagaagtgagtcttcacaccaagtctactttttgcaagttactgggtttctgtcttcaccatcttctgaaaagtctgcttctgttggttcagtttctggggtcatctgagtagagagattctgaaacagacactgatgttaatttgggggactacttttctcatgcaaacaggggagctcctagcaatcctgagaggtgctgcatccacatggtatgtggtgagacctttttgattaggaaataacagacacgtcctcataacattaaacaggttccacatcctactgtgcaattcccatctgaggacctggaaaactcaataggaggtcttaacagtggttgaacttgaagagtaagagctggatttcctggagtgtttctttgaggtgagggatacttgcatctgctttacagtgcggacacttcggcaaaggagagcgttctttgcatgatccctgaaatcatgtgaaacaaagtaatagacaaaggggtcgatgcagctgttaagggtagagaggcagagggctacaatgtacagggcatagacatggctctggccctggctcttaatcagaaaataatgcaccacaagcagaaggttactaggagtgaagcagatcaggtacatggccaggacagtgacaatgagtttgatggccctcttccttttcttctctgagttttcatccatggcagaagatcgcagcattctgatcatcagcacataggcagaggctgtgaggaaggctgggaacagaaagaccccaatggccagagagaggaagtaattgaacatgtctcccaccaagagctgctcaggcaaaacatcatgacaggtcgtgatgttcagggcaggaatgaagatggtctgcttcacgacatacaaaggaatggtgaccagcagaatcagcagccatattgccagggagatgccaatggcaatgtttgccttcttcctggagtgccccatggggttcacgatgacccaatacctctgcacactgaggcaggtcatgaagagaatggaacagtacatgttgccatagaaaaagccaataagcacattacaaagagcttccccataaatccagttgttgccatgtatgtgataggcaatcttcaaggggaaccagatgacagagaggaggtcagccaaggccagattggccatgtaaatcacagcagggtgcttcttcttagttcggaaaagaaagacccacagggccatgccgttacttggcaaacccaccacaaacacaattgtgtagacaattggaaggaagacagtggtcagttttccagtgaggacagatgcagaaaactcatccacagaaaagactgtttcaactgtaactccttttccagtgacgtgggatgtgccatcaaccttaccaataaggcttcttcctttagaggatctactggttccttggatggtgccactgcaggagagagaggctgctagcaggatggcggcccccagcagccacgccgcgctggggctccgcatcctcctggaagccccgacgccgggcgcgcggggaatccgccgccgccgattcgaaactcagagctccactggacgcaccgagagaaagtcagcctctcacctgccccgaatcggagcctctgctgcgcgcctccccagggcgggttaggtttc

SEQ ID NO: 19029 - RNA, 2137 nt, Homo sapiens
  source 1..2137: mol_type = other RNA
tggagtccaggaatctgcattttgaacaagattcacgactattttattttattttatcacccaagctggagtgcagtggtgcaatctcggctcactgcaacctctgcctcctgagttaaagtgatactcaattcttgtgcctcagcctcctgagtaactgggattacaaacgtgcaccacacacctggttaacttttgtatttttagtagagatgaggtttcgccatgatggccaggctggtctcgaactcctgacctcaagtgattgcctgcctcagcctcccaaagtgctaggattacaggcatgaggcaccgcacccagccaagatccatgattttgatgaagtggtacaagaacctcactcactggacattgaaattctactgtccaatcccaactcactgctgttgattggaaacctgattctggcagctcatttatcttggtttcctcatttgtaaggtcgttcagttggactgatcatctctgagggccttgaagccctaacaagtctatcatgatcccagatgtaaaatatatatatgtgtatatatataatttcagctgagaagtgagtcttcacaccaagtctactttttgcaagttactgggtttctgtcttcaccatcttctgaaaagtctgcttctgttggttcagtttctggggtcatctgagtagagagattctgaaacagacactgatgttaatttgggggactacttttctcatgcaaacaggggagctcctagcaatcctgagaggtgctgcatccacatggtatgtggtgagacctttttgattaggaaataacagacacgtcctcataacattaaacaggttccacatcctactgtgcaattcccatctgaggacctggaaaactcaataggaggtcttaacagtggttgaacttgaagagtaagagctggatttcctggagtgtttctttgaggtgagggatacttgcatctgctttacagtgcggacacttcggcaaaggagagcgttctttgcatgatccctgaaatcatgtgaaacaaagtaatagacaaaggggtcgatgcagctgttaagggtagagaggcagagggctacaatgtacagggcatagacatggctctggccctggctcttaatcagaaaataatgcaccacaagcagaaggttactaggagtgaagcagatcaggtacatggccaggacagtgacaatgagtttgatggccctcttccttttcttctctgagttttcatccatggcagaagatcgcagcattctgatcatcagcacataggcagaggctgtgaggaaggctgggaacagaaagaccccaatggccagagagaggaagtaattgaacatgtctcccaccaagagctgctcaggcaaaacatcatgacaggtcgtgatgttcagggcaggaatgaagatggtctgcttcacgacatacaaaggaatggtgaccagcagaatcagcagccatattgccagggagatgccaatggcaatgtttgccttcttcctggagtgccccatggggttcacgatgacccaatacctctgcacactgaggcaggtcatgaagagaatggaacagtacatgttgccatagaaaaagccaataagcacattacaaagagcttccccataaatccagttgttgccatgtatgtgataggcaatcttcaaggggaaccagatgacagagaggaggtcagccaaggccagattggccatgtaaatcacagcagggtgcttcttcttagttcggaaaagaaagacccacagggccatgccgttacttggcaaacccaccacaaacacaattgtgtagacaattggaaggaagacagtggtcagttttccagtgaggacagatgcagaaaactcatccacagaaaagactgtttcaactgtaactccttttccagtgacgtgggatgtgccatcaaccttaccaataaggcttcttcctttagaggatctactggttcctttgctcctgaattttaagtttccaactttaaaggacatagaggagaggtgtccattacagttttcaatacttcctggaactaaatgcctttattctgatgctgattaagaaaaaaaaatataccagcggtgcacagttt

SEQ ID NO: 19030 - RNA, 165 nt, Homo sapiens
  source 1..165: mol_type = other RNA
tggagtccaggaatctgcatttttaaaatcagcctaagtatgttctaatgcctgaacacacttctaaagcctgcaaaacacttataaaccggtgtttccactgggtgtggtggctcatgtctgtaatcctagcactttgggaggccaaggcaggtggatggcttg

SEQ ID NO: 19031 - RNA, 308 nt, Homo sapiens
  source 1..308: mol_type = other RNA
tggagtccaggaatctgcatttttaaacatatccattagagatcttgaagtgttcctaggattcattaattccatgcatactgaataaatcctcctgtgtaccaggcactttgagatgctgaggggacagcagtgaacaatttagacaaggctactgctctcctggtgcttacattttaatgtgaaacaaagaaaggaggatacttgacatcaatatgtgatacaaagtaaataaaacgggatattaagatagaaagtcaggagctggacacaatggcttgtgcctgtaatcctagcactttgggagg

SEQ ID NO: 19032 - RNA, 852 nt, Homo sapiens
  source 1..852: mol_type = other RNA
tggagtccaggaatctgcatttttaacaaagtttgagaactggtgctagggaatgtgaccactctactattttagttgtgacacttaattcagatactcccattaagtgaatatcaaaatctttagataatatttaatttcaaaatttctcccttctgagggaccacttaatatattaattcagagggcttacttaattcatctttttattgttatatatattgccttgaaaaggaaaggtcttaattatatacagaatacaatatatgaggctgggtgtgatggctcatgcctgtaatcctagcactttgggaagtcgaggcgggcagctctcttgaggtcaggagttcgaaatcagcctggccaacatgatgaaaccccgtatctactgggaggtggaggttgcagtgagccaagatcacaccattgcactccagcctgggcaacaagagggagactccattgtgattacgtgattcactttccagaatgaggcacacttcaaagttgactcatcggcaaaatcaggtgagccaggttctaagacagtgctttcctgctggcaggcatcaagacgaagacaggcagccattgttggggagggagtcgacatcaagctggtatctcatctagctcgtgacttttctatactgagcaccttccaggtgtccaggtgagaacacaacatggataaggcttactttacatctgtcagagccctggcaaatgccttcccgagtgcctctggcattctctgtgagaaagagagccacagcctgacaactcccatagccatcaatggcaacgctcctgaccctcaagacattccaaaaggattaaaaccaagagcaa

SEQ ID NO: 19033 - RNA, 2860 nt, Homo sapiens
  source 1..2860: mol_type = other RNA
tggagtccaggaatctgcatttttaacaaggtccctaggagactctgatgcaggtggtgtagaccacatgctttaggaaggagaaacagcttctgacctgtttactcctgtctctccagcatgataaacacaatgctagttacacatgcaatatgtatttgttgaattacttgtttaatgcatacaataaatatttgtcaaattgtttaatcatgcttcactctatagcattttagagtttataaaacattctatgtgctttatatgatgattcccaaatctatatataaaccaggccatccactaaagctcatatttcatctttaaacagctctattgagcatttttacctgtatatttcagaaatctcaacatatctaaaaaccatattcattatttttcaggcaaagccactttctcgaatttccttattttctcaaccatgacattattttctaagtcatccttgacttctttctctcattcacctctgtatgctaaattctgctgaattttgttttgaaaacttcttccttgcccccagagctcatctttatttctgctgcagcagccctagctcaggcgtttatcagctgcctcctaaactattagaatggaatcttagctacctctctcctaagttactagatcaattgctagatcacattttctaacatatatactttaccatattatccttttacataaaaactttaatactatccacagtctctgaagaatagagcccagttcctctgtctggcacccaaaacactccactatgacactggcgtttataatttcagcctcatcacccactgccccctgttggaatcctgttctcccctgagacttccctctgaatgcaccctacttatttataaggctgaacaactgctccatccccctgctcccatcattaatatggaaaggaatcaagaccctaatttgggacttactctttccaggtaggctaaggttcttacttggttggaagaagattataaaacaaggatgtaggtgggaccatgatggttttgggggctcttatatcccttttctctttcactcttccccaactctcttgacagtccttctcattgactgcatgtgggtttgctgttttcacatcaatatgccaaagagaaaaggtggttggggtttctctctggaaacttacctgcgatgggtgggctcaccaagtatggcactgcgtgaaggaagtataccacaccaagcgctgatgacaaagaggtggtccccactatctctgtggtcactactgggatcaaagtcacataggcaccatcaaagtagccaaaggtacaagagaaaggcacgagcagagggagactttgaagcattgggaggcagagatagcagagcccatccattcccacggcaaagaggtagcaaacatactggtaattcttcagacaccttctgtcggtcagccatccaaatgtgatattgccaataatgtcaatcactccaagtatggacataagaaaagcagcttgctgatgactcactccaacactcaaagcataaggcaccaagtacacaaagagagggctgcagccataagccataaacagaacggagacggctaacacaacaaagtctgacatgagtaaaaaactgtactcttgctgcaaacagcaacagaggcaagtctgtgcccattctttggtcaaagatgaatagggagacacccgcttaatgtcttctttctgagttctacacacatggttctgctctggagttgtgtggtcctctttaagagtaattggcctcatcaaggcaccacatacacagagattcaagacaaagcccccaagaatgagtaaggctccccgccaggaaaactgttcaataaggagctgaaccacaggagccaggatgaaggtgccaatgccacttcctgacatggcgataccataagcaagggctttccgtctgctgaagtacttgccaaccatggcaatagctggagagtaacaaagtgcaaatccaagacctgtaagaactcccagagtgaggtagagatgcttcagactcgtggcaaatgagctcaggatgagtccagtagatgcaagcaagccacccagcatgattcccacttgacaggataaatggttactgacaacactcccaagtggagcacagagcatggtcacacaatctacaatggaatggatccatgccgtttgtgcgtaatcctgagtgaagtatgtctggaactccacaaaaaaaattgagatacatcttgtgactgcccgtgtgcagatggtaacaaggaaacagccagccacaatcatccagccccagcctccatctggaggggaggtagaccgagctctatttacttttgccatggtttttcttttttcttcttttccaggttgctccaacagccaagttatgatcttggaagagtttgctgtccagtgacttcctgatggcattcaaggttggcatagaacgctacctggcccatgggttactcgccatctcgccgggaccactgcagccctggcggtagcgcgcggacatgcccccggggcgcacccgccgagccgcgtccctgcgcagtggccccttcccgggccccaggctgcgcgatccgcgcttcggtggggcggggagcggactgggcggaggcgccggcgaggctggggccgggggcctagctggcaacgccgggagagggaagcgtagcgcggaaaatcccagtgctcggccttcgaaatgcaccggctcattcagccccgccagctccgccggggactctgcctggccggcaaagaggatttagcgcggggatccgctctaagtactgtggcttggctaggggcga

SEQ ID NO: 19034 - RNA, 56 nt, Homo sapiens
  source 1..56: mol_type = other RNA
tggagtccaggaatctgcatttttaaccagctgccctggcaattctgacacacact

SEQ ID NO: 19035 - RNA, 60 nt, Homo sapiens
  source 1..60: mol_type = other RNA
tggagtccaggaatctgcatttttaaccagctgccctggcaattctgacacacactaact

SEQ ID NO: 19036 - RNA, 6653 nt, Homo sapiens
  source 1..6653: mol_type = other RNA
tggagtccaggaatctgcatttttacaagtgctacacatgatttttgtgcatactgagtattaaaaaacactattaaaaagtttgcaatggagatcactggaaaaagaatctccattccaacgtatacagcaagatgagaataataggcatttcaaacaaataagctctgtgtttgcatcacaaggctgtgattattaaagtttaagactctattctttcagcaggggtagagagcaataaccatttcgtctgaaaccagaatgatgaaggcaatataaatcaaacctattccagcaggtttcatttggtctaatttctctgcagatattaatcattatacagttctatacaaatgacatgtaactccattgtaactcaggatacagaatgttcactctggttctttctctagtgtgctattttgacaatataaaagaaaataaataaattgaaactgtggggcatcaagattgcaagacaccaacaataccaagacattaaagagagaaatggcccatgctaaacctataaaccagcatgcaaattggcaaaaacatttatctgccacagagtcaccataaggaaaaataaactcccttcgtttttcttttgaaaattggtatgtcaggtggaggtgacaaagaattcttcctaaaagttcacagaaagagtattattaattctagtaaagatcatctagaagaccaaggctagtcaaattccatggcatggtatatagtggcagaaaataccagcactcaaattcacagatctacactatagtagatacaaagttgaaggttggaattgtagcaaaggaaaatgtataagaatcaaaatttggttcccattgtgggagctggtgtcaagtaattttacaaaacaccatacatgccttccttttgtctcattgtaacatgttttgtctgacaccaacaaaggatcctcagagaagaatctaaagcccaggaaagcaaaagtaatccagaagcgcaggcagtaatggggcccagaacaagcaacacacctgtgcctatggataaagattcctctgaatctaacaaggctaattgaaaagagaaaaattccatgtcaacatcccttaataaatgtgttcccccaaaatgaattggttggaatagatacaactataaaggaataaagagcaaagggaacgcttattatttgtgcattgttcccccttttattttaattcaccatgcatgcattttcagtaagataactgtgcctataaatacaaaggataacatcagtgcatattttggaagccacttcatttcattattttttgtcagcatttcagtgcaattttttcctagcaggggaaagaaaatcacaataccatatgatctagtagttttacattcctgtcttccccttttcctgctgaatgcagatcagttcatttttgatagtgggtagaaggactttgtaaatatgtttctgacttcagacaacccacatacctttagggaatgatctcccaaagctcactggattttagtatcgcgggatttcccagaaggcaatctaagttggggctctacacatgtgattccccattcattgtatccactcaatactactaacttctttatattagcaatttatggcccttgtcataaccaatgttcgagaagtaaaccatatatattgttttcttcagaattaaacaaaaagttctaaaaactattttaacttcagggaaacatgcccgagtcacagtgactaccagagttactagagcatgtactcttataactcacttacccagaactcatttccagtgttgcaggctacctggacctcacttgataactccactcaaactaggtactttaagcctcctcagagccttttactggccaggtctatgttcatttctatataaacactcacacaaataaatgccatgctgttgtcttagttacttgaatattttaccatgggatgagtgccagtcgagaggtggcccagaataaaaatattgctgttgtgatggttttaaacaggttttctattccagctttgttcactggatgtataaggaatgtcagagcagagaaaactcatgacaggtcaggggtcagaggaacactgccacgaacactccttttgcagtgtttaatttcctgtttaaagaatgtagtagaaatattgggttgactatcatcttaattctttactcttataagggtatctctctatcttgaggccattacagtcaggtctgaaatttaaggaagttggaactttggccattttagttagacccccaaagtctttgacagtacttccagtgacaacacaataatcatttgaccaaagtgagtttcaggatattttccccaaattcaacttcttgacccattaagctctgtgattctttgcaagatcttctgttattaggatgatggtattgccatgtgctatcaagaaacattgaaaagaatcaagacatactggtaagtttacaaacaaagctatgttgtagttaagaccaaatatctgctaatatattaatacagaaaagaataccacttaaattcataaattataattctcttgacaactcaactcccaagataaactttctttttcacttatgtaaaactttcaactccattcaaaccttcaggacaaggaaacattagctgagtctgtcatcctagtgtgaaggcgagaattacaaaaattcagaaagatattcatatactaatcatcactaagaacagaaatcaagacagaacatcttacataataaatgtgcatcaatgaaagatttcaaaaggaagaaattagtcattgttttcctcctacagatatcatccaattgcctttattacctgtgatacacatacacacatgcacacacacgcaataaaacaaattaggagtgcttggcacacaactattaattgacaaattattttttggttaccactgaaatgcatgaggaatgctgaaaataaaactggtcttttaaccttcttgtagcacaagtctatgaaagagctattggtaccttagtaaaatacagagttacatggacggatggctattaacagtttctttttggctgtgtctatacaagtcaggatgtaattgaaaaagatagtttcatttagaaatctgaaaccttaactctggagcttcagttaccttgttgggttgttacagacatcataaaaatgacacagctaaatcctagcatgggcacagccaaagcccgaatcccaaaggcaaacaaaaacggctacaagcaagtaaaaatgtagctttgtagtttaaaatttttataagaaattattaggttgtgtgtggaatacaactttctctaaaacaaacaaaaggccggacccttattcaagtactgtgtgttgtccttagttccacaacaacacaggaacacagaacttaatgtggattatgtggaaaggccacaccattaaactgtgggcagtaagaactctgaaaacatggagaaaagggtgataattcagttcagggtagagaaggctgagtgtggagtcatttagcagaaaattttgtggatatgaatgtttgatttttttaacacaaggaatgtttgaccagctctcctcatcctctcttaatgcagacaaagagcaaagcagtaaaatggagcctgagggtattaatttcacaataaggaatacaatttgttgatgatgagagtcatttgatgttagaaagtgttgtgaagaaaggctgggaaatcttcccaaaagaattttaagaaagagtcagaagctcatccatctgaaatattctaagagagggctgctgggagcaggagcacagcccttgggaggtctaggccctggcatcgtgtgcgtcatgtgtatatacatacttagttgtgcttgtgttgcacaaatactcatgcatacggagtcaatataaactggcacatatagatttgagtgaaaagtcatataaatctgccattccccccaaccccataaacaaaaggaaaaaccaaaattaaaaattccaaacttatgccattgggccagatctttttctaccataccctcattcaaaggagggaggtagaaggatgagagaaaaaacccagtttgggataaatgactcccaaggcctctcagctacttttacgtagctggctctcattatatataagatagttagcacatgggacgaagtaaacaaacaaataactaaaaaagattttcttgtacttccacatctagaaagaaatctaccctgtggatttacatgttaaggtgaactaggtaaagtaggcagtagtatatcaatggactattgtgttctaagaaatgtgcatcattagttgtatttttttcctttaaaatatgaattccttttaggaggttaatttcaaaatgacttttttttttcttttcccgcccccagccctcccttatagatgatacttccttaaaagttcagattgccaaggatgttttctctcaggaaaccgatctggaattttgatttttaggaaatcctggatacatttctccagctcctcctcaattgagagcttttctttaacagctttttttttgctgctcatgttcgattccctggagcctgaagtcagagtccggagtaagtcgcttttccgccgcatctctgactgttggatcagctggacagggcccttcttgatgggacggtccagagtctggatgttggtctggcgtgtcacgggaccacagatgaccgtctcctggggagagctggcctcagactggctgtcgcagctagatgtggagaggtcattgcaagacgtgccgctctccccttctttgtcacctttgccattcttgcagcagcaatcgcagtgtgagggtgaccatctggaaggctcacggtagaagacatattcagtgtagcttgaccagatcttgtcatctgtatattggttgatgaaagatgctgtcaccgatgagttacaggccaccatgtggaatccacactctgacaacatatcaaaagccctttccaggtgcttgaatttgagataaaatctggaggtgtatctttctggggctcgatcagggtctctgctttcattcaaagtttctccaaagacttcttttgccaaggaaatccttccacaaaccaaaatccggggaactctccgaaacttggcatctgcctgtccctctctgcccaaggtgcaggatcctctgtaacccacagtaatgaaaccccacttgcggtcggcagggagcagggaggaaggggggcagattcttgtgtcgcttccttgggaggcatcttcaaagtcactgtggcagaattcatctgggctttgcttgatttcatcgggggtcaggagtttgaccaagtctgggagctggaagtattcagcttcccttttcagtcttcctttttctggaaagtgatcaggcaggaccacctgcctgtccctgagatagtccagaatataacggaacaagaatccatctctgtcaatgaaaaaccttcccttggagtccttggctagatcattagccgtgtctctctttggggaaaacattttccacaggagggaatgagggatgcttatcaatgtggaatggcgagtaaaataaacttgacccccgacattcagctctaccacctcagggaaggagttgggaactgcggacccttgttctcgaggataataacgactacagtttccactcagagccattgtccctttcttctgctgctgctattttgatttaaaggtgcaatccaatggagtcacagccttatcctttggatcaacttgtaagaaagggaaaaggatgctaacttattaaaaaatgacctcctcttatcccagtatttttcccccaagaaatcaaaatgtataagagtccacaggtgaagtgatgctgaaaaagtagtttaaaccctggatggtggatggtagtgagctgctacttcataaaatataatcaactcgtctatatccaatcttccatcaagctcacatgcaaggcaggccaattccccagttactcagatgtccgtaacgaatctgcagttccctccaaaaccttttccggtggatttccccagtctgtcttcacaggttgtgggttgtcagcctcatcctgaatgcaataagtagttctgacacagaggccacataaactctttaaagccaattggtttttaccattattgtcaggtttcattgtggaacttgactgaaatacacagagctgccagatctccacttcatgtgatgcttgtggatatagctgacggtaggagaaaactgcccatgttcaaaccataattttctggcacaacttttcatgacatatgaaaaacactttagcacagtgcttgaatcacagtaaatgctgacaccgaggcattgtaggcattgtagtttgtggacaggagaggggactccgtctgtctcattttagcgcctcccagtcttcctccatcacctaggtctgagaaactcctcctcctacctacgagtaagcagcaattgctacgcctgcgctttcctggttccacccctaaccaggctgccggaagcactttcctctttggcacgggccagccgcaggttgggtagatactgcgcaagctccatactcgt

SEQ ID NO: 19037 - RNA, 6367 nt, Homo sapiens
  source 1..6367: mol_type = other RNA
tggagtccaggaatctgcatttttacaagtgctacacatgatttttgtgcatactgagtattaaaaaacactattaaaaagtttgcaatggagatcactggaaaaagaatctccattccaacgtatacagcaagatgagaataataggcatttcaaacaaataagctctgtgtttgcatcacaaggctgtgattattaaagtttaagactctattctttcagcaggggtagagagcaataaccatttcgtctgaaaccagaatgatgaaggcaatataaatcaaacctattccagcaggtttcatttggtctaatttctctgcagatattaatcattatacagttctatacaaatgacatgtaactccattgtaactcaggatacagaatgttcactctggttctttctctagtgtgctattttgacaatataaaagaaaataaataaattgaaactgtggggcatcaagattgcaagacaccaacaataccaagacattaaagagagaaatggcccatgctaaacctataaaccagcatgcaaattggcaaaaacatttatctgccacagagtcaccataaggaaaaataaactcccttcgtttttcttttgaaaattggtatgtcaggtggaggtgacaaagaattcttcctaaaagttcacagaaagagtattattaattctagtaaagatcatctagaagaccaaggctagtcaaattccatggcatggtatatagtggcagaaaataccagcactcaaattcacagatctacactatagtagatacaaagttgaaggttggaattgtagcaaaggaaaatgtataagaatcaaaatttggttcccattgtgggagctggtgtcaagtaattttacaaaacaccatacatgccttccttttgtctcattgtaacatgttttgtctgacaccaacaaaggatcctcagagaagaatctaaagcccaggaaagcaaaagtaatccagaagcgcaggcagtaatggggcccagaacaagcaacacacctgtgcctatggataaagattcctctgaatctaacaaggctaattgaaaagagaaaaattccatgtcaacatcccttaataaatgtgttcccccaaaatgaattggttggaatagatacaactataaaggaataaagagcaaagggaacgcttattatttgtgcattgttcccccttttattttaattcaccatgcatgcattttcagtaagataactgtgcctataaatacaaaggataacatcagtgcatattttggaagccacttcatttcattattttttgtcagcatttcagtgcaattttttcctagcaggggaaagaaaatcacaataccatatgatctagtagttttacattcctgtcttccccttttcctgctgaatgcagatcagttcatttttgatagtgggtagaaggactttgtaaatatgtttctgacttcagacaacccacatacctttagggaatgatctcccaaagctcactggattttagtatcgcgggatttcccagaaggcaatctaagttggggctctacacatgtgattccccattcattgtatccactcaatactactaacttctttatattagcaatttatggcccttgtcataaccaatgttcgagaagtaaaccatatatattgttttcttcagaattaaacaaaaagttctaaaaactattttaacttcagggaaacatgcccgagtcacagtgactaccagagttactagagcatgtactcttataactcacttacccagaactcatttccagtgttgcaggctacctggacctcacttgataactccactcaaactaggtactttaagcctcctcagagccttttactggccaggtctatgttcatttctatataaacactcacacaaataaatgccatgctgttgtcttagttacttgaatattttaccatgggatgagtgccagtcgagaggtggcccagaataaaaatattgctgttgtgatggttttaaacaggttttctattccagctttgttcactggatgtataaggaatgtcagagcagagaaaactcatgacaggtcaggggtcagaggaacactgccacgaacactccttttgcagtgtttaatttcctgtttaaagaatgtagtagaaatattgggttgactatcatcttaattctttactcttataagggtatctctctatcttgaggccattacagtcaggtctgaaatttaaggaagttggaactttggccattttagttagacccccaaagtctttgacagtacttccagtgacaacacaataatcatttgaccaaagtgagtttcaggatattttccccaaattcaacttcttgacccattaagctctgtgattctttgcaagatcttctgttattaggatgatggtattgccatgtgctatcaagaaacattgaaaagaatcaagacatactggtaagtttacaaacaaagctatgttgtagttaagaccaaatatctgctaatatattaatacagaaaagaataccacttaaattcataaattataattctcttgacaactcaactcccaagataaactttctttttcacttatgtaaaactttcaactccattcaaaccttcaggacaaggaaacattagctgagtctgtcatcctagtgtgaaggcgagaattacaaaaattcagaaagatattcatatactaatcatcactaagaacagaaatcaagacagaacatcttacataataaatgtgcatcaatgaaagatttcaaaaggaagaaattagtcattgttttcctcctacagatatcatccaattgcctttattacctgtgatacacatacacacatgcacacacacgcaataaaacaaattaggagtgcttggcacacaactattaattgacaaattattttttggttaccactgaaatgcatgaggaatgctgaaaataaaactggtcttttaaccttcttgtagcacaagtctatgaaagagctattggtaccttagtaaaatacagagttacatggacggatggctattaacagtttctttttggctgtgtctatacaagtcaggatgtaattgaaaaagatagtttcatttagaaatctgaaaccttaactctggagcttcagttaccttgttgggttgttacagacatcataaaaatgacacagctaaatcctagcatgggcacagccaaagcccgaatcccaaaggcaaacaaaaacggctacaagcaagtaaaaatgtagctttgtagtttaaaatttttataagaaattattaggttgtgtgtggaatacaactttctctaaaacaaacaaaaggccggacccttattcaagtactgtgtgttgtccttagttccacaacaacacaggaacacagaacttaatgtggattatgtggaaaggccacaccattaaactgtgggcagtaagaactctgaaaacatggagaaaagggtgataattcagttcagggtagagaaggctgagtgtggagtcatttagcagaaaattttgtggatatgaatgtttgatttttttaacacaaggaatgtttgaccagctctcctcatcctctcttaatgcagacaaagagcaaagcagtaaaatggagcctgagggtattaatttcacaataaggaatacaatttgttgatgatgagagtcatttgatgttagaaagtgttgtgaagaaaggctgggaaatcttcccaaaagaattttaagaaagagtcagaagctcatccatctgaaatattctaagagagggctgctgggagcaggagcacagcccttgggaggtctaggccctggcatcgtgtgcgtcatgtgtatatacatacttagttgtgcttgtgttgcacaaatactcatgcatacggagtcaatataaactggcacatatagatttgagtgaaaagtcatataaatctgccattccccccaaccccataaacaaaaggaaaaaccaaaattaaaaattccaaacttatgccattgggccagatctttttctaccataccctcattcaaaggagggaggtagaaggatgagagaaaaaacccagtttgggataaatgactcccaaggcctctcagctacttttacgtagctggctctcattatatataagatagttagcacatgggacgaagtaaacaaacaaataactaaaaaagattttcttgtacttccacatctagaaagaaatctaccctgtggatttacatgttaaggtgaactaggtaaagtaggcagtagtatatcaatggactattgtgttctaagaaatgtgcatcattagttgtatttttttcctttaaaatatgaattccttttaggaggttaatttcaaaatgacttttttttttcttttcccgcccccagccctcccttatagatgatacttccttaaaagttcagattgccaaggatgttttctctcaggaaaccgatctggaattttgatttttaggaaatcctggatacatttctccagctcctcctcaattgagagcttttctttaacagctttttttttgctgctcatgttcgattccctggagcctgaagtcagagtccggagtaagtcgcttttccgccgcatctctgactgttggatcagctggacagggcccttcttgatgggacggtccagagtctggatgttggtctggcgtgtcacgggaccacagatgaccgtctcctggggagagctggcctcagactggctgtcgcagctagatgtggagaggtcattgcaagacgtgccgctctccccttctttgtcacctttgccattcttgcagcagcaatcgcagtgtgagggtgaccatctggaaggctcacggtagaagacatattcagtgtagcttgaccagatcttgtcatctgtatattggttgatgaaagatgctgtcaccgatgagttacaggccaccatgtggaatccacactctgacaacatatcaaaagccctttccaggtgcttgaatttgagataaaatctggaggtgtatctttctggggctcgatcagggtctctgctttcattcaaagtttctccaaagacttcttttgccaaggaaatccttccacaaaccaaaatccggggaactctccgaaacttggcatctgcctgtccctctctgcccaaggtgcaggatcctctgtaacccacagtaatgaaaccccacttgcggtcggcagggagcagggaggaaggggggcagattcttgtgtcgcttccttgggaggcatcttcaaagtcactgtggcagaattcatctgggctttgcttgatttcatcgggggtcaggagtttgaccaagtctgggagctggaagtattcagcttcccttttcagtcttcctttttctggaaagtgatcaggcaggaccacctgcctgtccctgagatagtccagaatataacggaacaagaatccatctctgtcaatgaaaaaccttcccttggagtccttggctagatcattagccgtgtctctctttggggaaaacattttccacaggagggaatgagggatgcttatcaatgtggaatggcgagtaaaataaacttgacccccgacattcagctctaccacctcagggaaggagttgggaactgcggacccttgttctcgaggataataacgactacagtttccactcagagccattgtccctttcttctgctgctgctattttgatttaaaggtgcaatccaatggagtcacagccttatcctttggatcaacttgtaagaaagggaaaaggatgctaacttattaaaaaatgacctcctcttatcccagtatttttcccccaagaaatcaaaatgtataagagtccacaggtgaagtgatgctgaaaaagtagtttaaaccctggatggtggatggtagtgagctgctacttcataaaatataatcaactcgtctatatccaatcttccatcaagctcacatgcaaggcaggccaattccccagttactcagatgtccgtattggtttttaccattattgtcaggtttcattgtggaacttgactgaaatacacagagctgccagatctccacttcatgtgatgcttgtggatatagctgacggtaggagaaaactgcccatgttcaaaccataattttctggcacaacttttcatgacatatgaaaaacactttagcacagtgcttgaatcacagtaaatgctgacaccgaggcattgtaggcattgtagtttgtggacaggagaggggactccgtctgtctcattttagcgcctcccagtcttcctccatcacctaggtct

SEQ ID NO: 19038 - RNA, 6775 nt, Homo sapiens
  source 1..6775: mol_type = other RNA
tggagtccaggaatctgcatttttacaagtgctacacatgatttttgtgcatactgagtattaaaaaacactattaaaaagtttgcaatggagatcactggaaaaagaatctccattccaacgtatacagcaagatgagaataataggcatttcaaacaaataagctctgtgtttgcatcacaaggctgtgattattaaagtttaagactctattctttcagcaggggtagagagcaataaccatttcgtctgaaaccagaatgatgaaggcaatataaatcaaacctattccagcaggtttcatttggtctaatttctctgcagatattaatcattatacagttctatacaaatgacatgtaactccattgtaactcaggatacagaatgttcactctggttctttctctagtgtgctattttgacaatataaaagaaaataaataaattgaaactgtggggcatcaagattgcaagacaccaacaataccaagacattaaagagagaaatggcccatgctaaacctataaaccagcatgcaaattggcaaaaacatttatctgccacagagtcaccataaggaaaaataaactcccttcgtttttcttttgaaaattggtatgtcaggtggaggtgacaaagaattcttcctaaaagttcacagaaagagtattattaattctagtaaagatcatctagaagaccaaggctagtcaaattccatggcatggtatatagtggcagaaaataccagcactcaaattcacagatctacactatagtagatacaaagttgaaggttggaattgtagcaaaggaaaatgtataagaatcaaaatttggttcccattgtgggagctggtgtcaagtaattttacaaaacaccatacatgccttccttttgtctcattgtaacatgttttgtctgacaccaacaaaggatcctcagagaagaatctaaagcccaggaaagcaaaagtaatccagaagcgcaggcagtaatggggcccagaacaagcaacacacctgtgcctatggataaagattcctctgaatctaacaaggctaattgaaaagagaaaaattccatgtcaacatcccttaataaatgtgttcccccaaaatgaattggttggaatagatacaactataaaggaataaagagcaaagggaacgcttattatttgtgcattgttcccccttttattttaattcaccatgcatgcattttcagtaagataactgtgcctataaatacaaaggataacatcagtgcatattttggaagccacttcatttcattattttttgtcagcatttcagtgcaattttttcctagcaggggaaagaaaatcacaataccatatgatctagtagttttacattcctgtcttccccttttcctgctgaatgcagatcagttcatttttgatagtgggtagaaggactttgtaaatatgtttctgacttcagacaacccacatacctttagggaatgatctcccaaagctcactggattttagtatcgcgggatttcccagaaggcaatctaagttggggctctacacatgtgattccccattcattgtatccactcaatactactaacttctttatattagcaatttatggcccttgtcataaccaatgttcgagaagtaaaccatatatattgttttcttcagaattaaacaaaaagttctaaaaactattttaacttcagggaaacatgcccgagtcacagtgactaccagagttactagagcatgtactcttataactcacttacccagaactcatttccagtgttgcaggctacctggacctcacttgataactccactcaaactaggtactttaagcctcctcagagccttttactggccaggtctatgttcatttctatataaacactcacacaaataaatgccatgctgttgtcttagttacttgaatattttaccatgggatgagtgccagtcgagaggtggcccagaataaaaatattgctgttgtgatggttttaaacaggttttctattccagctttgttcactggatgtataaggaatgtcagagcagagaaaactcatgacaggtcaggggtcagaggaacactgccacgaacactccttttgcagtgtttaatttcctgtttaaagaatgtagtagaaatattgggttgactatcatcttaattctttactcttataagggtatctctctatcttgaggccattacagtcaggtctgaaatttaaggaagttggaactttggccattttagttagacccccaaagtctttgacagtacttccagtgacaacacaataatcatttgaccaaagtgagtttcaggatattttccccaaattcaacttcttgacccattaagctctgtgattctttgcaagatcttctgttattaggatgatggtattgccatgtgctatcaagaaacattgaaaagaatcaagacatactggtaagtttacaaacaaagctatgttgtagttaagaccaaatatctgctaatatattaatacagaaaagaataccacttaaattcataaattataattctcttgacaactcaactcccaagataaactttctttttcacttatgtaaaactttcaactccattcaaaccttcaggacaaggaaacattagctgagtctgtcatcctagtgtgaaggcgagaattacaaaaattcagaaagatattcatatactaatcatcactaagaacagaaatcaagacagaacatcttacataataaatgtgcatcaatgaaagatttcaaaaggaagaaattagtcattgttttcctcctacagatatcatccaattgcctttattacctgtgatacacatacacacatgcacacacacgcaataaaacaaattaggagtgcttggcacacaactattaattgacaaattattttttggttaccactgaaatgcatgaggaatgctgaaaataaaactggtcttttaaccttcttgtagcacaagtctatgaaagagctattggtaccttagtaaaatacagagttacatggacggatggctattaacagtttctttttggctgtgtctatacaagtcaggatgtaattgaaaaagatagtttcatttagaaatctgaaaccttaactctggagcttcagttaccttgttgggttgttacagacatcataaaaatgacacagctaaatcctagcatgggcacagccaaagcccgaatcccaaaggcaaacaaaaacggctacaagcaagtaaaaatgtagctttgtagtttaaaatttttataagaaattattaggttgtgtgtggaatacaactttctctaaaacaaacaaaaggccggacccttattcaagtactgtgtgttgtccttagttccacaacaacacaggaacacagaacttaatgtggattatgtggaaaggccacaccattaaactgtgggcagtaagaactctgaaaacatggagaaaagggtgataattcagttcagggtagagaaggctgagtgtggagtcatttagcagaaaattttgtggatatgaatgtttgatttttttaacacaaggaatgtttgaccagctctcctcatcctctcttaatgcagacaaagagcaaagcagtaaaatggagcctgagggtattaatttcacaataaggaatacaatttgttgatgatgagagtcatttgatgttagaaagtgttgtgaagaaaggctgggaaatcttcccaaaagaattttaagaaagagtcagaagctcatccatctgaaatattctaagagagggctgctgggagcaggagcacagcccttgggaggtctaggccctggcatcgtgtgcgtcatgtgtatatacatacttagttgtgcttgtgttgcacaaatactcatgcatacggagtcaatataaactggcacatatagatttgagtgaaaagtcatataaatctgccattccccccaaccccataaacaaaaggaaaaaccaaaattaaaaattccaaacttatgccattgggccagatctttttctaccataccctcattcaaaggagggaggtagaaggatgagagaaaaaacccagtttgggataaatgactcccaaggcctctcagctacttttacgtagctggctctcattatatataagatagttagcacatgggacgaagtaaacaaacaaataactaaaaaagattttcttgtacttccacatctagaaagaaatctaccctgtggatttacatgttaaggtgaactaggtaaagtaggcagtagtatatcaatggactattgtgttctaagaaatgtgcatcattagttgtatttttttcctttaaaatatgaattccttttaggaggttaatttcaaaatgacttttttttttcttttcccgcccccagccctcccttatagatgatacttccttaaaagttcagattgccaaggatgttttctctcaggaaaccgatctggaattttgatttttaggaaatcctggatacatttctccagctcctcctcaattgagagcttttctttaacagctttttttttgctgctcatgttcgattccctggagcctgaagtcagagtccggagtaagtcgcttttccgccgcatctctgactgttggatcagctggacagggcccttcttgatgggacggtccagagtctggatgttggtctggcgtgtcacgggaccacagatgaccgtctcctggggagagctggcctcagactggctgtcgcagctagatgtggagaggtcattgcaagacgtgccgctctccccttctttgtcacctttgccattcttgcagcagcaatcgcagtgtgagggtgaccatctggaaggctcacggtagaagacatattcagtgtagcttgaccagatcttgtcatctgtatattggttgatgaaagatgctgtcaccgatgagttacaggccaccatgtggaatccacactctgacaacatatcaaaagccctttccaggtgcttgaatttgagataaaatctggaggtgtatctttctggggctcgatcagggtctctgctttcattcaaagtttctccaaagacttcttttgccaaggaaatccttccacaaaccaaaatccggggaactctccgaaacttggcatctgcctgtccctctctgcccaaggtgcaggatcctctgtaacccacagtaatgaaaccccacttgcggtcggcagggagcagggaggaaggggggcagattcttgtgtcgcttccttgggaggcatcttcaaagtcactgtggcagaattcatctgggctttgcttgatttcatcgggggtcaggagtttgaccaagtctgggagctggaagtattcagcttcccttttcagtcttcctttttctggaaagtgatcaggcaggaccacctgcctgtccctgagatagtccagaatataacggaacaagaatccatctctgtcaatgaaaaaccttcccttggagtccttggctagatcattagccgtgtctctctttggggaaaacattttccacaggagggaatgagggatgcttatcaatgtggaatggcgagtaaaataaacttgacccccgacattcagctctaccacctcagggaaggagttgggaactgcggacccttgttctcgaggataataacgactacagtttccactcagagccattgtccctttcttctgctgctgctattttgatttaaaggtgcaatccaatggagtcacagccttatcctttggatcaacttgtaagaaagggaaaaggatgctaacttattaaaaaatgacctcctcttatcccagtatttttcccccaagaaatcaaaatgtataagagtccacaggtgaagtgatgctgaaaaagtagtttaaaccctggatggtggatggtagtgagctgctacttcataaaatataatcaactcgtctatatccaatcttccatcaagctcacatgcaaggcaggccaattccccagttactcagatgtccgtctgaaggaaaagagaaaaaattatttcctcaaacctggaatgagtcagaaaaagagtcctcttagtgagtgctggagacccagttcttgtgaaaaaaataataataaccatttgtaaagcaatcaaaatccacagccaaactgagtctggatcttgtcaaatcccaaacaggtaaacgaccgaggtatcaatgaaaagtgccagagaggtgtgctcttggaaaataactattatatatatgcatttatataaatgcctatttgtatttatgtatgtatgtaggtacatatgtgttcattccgtatcttaagttaaaacaagtcgcaaaaaaagttaagccctgatgagaggaggttgggttgaagaagtaaagcagagaaaatattcaaccaaagcttccccaggggaaaagaaaaatggaaaaagaaatctttggaaaggatccttagaagagagttgcaagaggtaccaggacttagaagcttttcagaaagcccagaagcagaaagatggagagatgtgccctgctagggtcccaggtagccaccccacctgccggcaagggcaaacggactcccatgttcccagccaggtgggagccggtgcgagccagaggccaacgcagcgcagagatgccggcggggggcccggggctccggcttctctggcggcggagctgggtggttccacagttcccagtgcagttcggat

SEQ ID NO: 19039 - RNA, 6154 nt, Homo sapiens
  source 1..6154: mol_type = other RNA
tggagtccaggaatctgcatttttacaagtgctacacatgatttttgtgcatactgagtattaaaaaacactattaaaaagtttgcaatggagatcactggaaaaagaatctccattccaacgtatacagcaagatgagaataataggcatttcaaacaaataagctctgtgtttgcatcacaaggctgtgattattaaagtttaagactctattctttcagcaggggtagagagcaataaccatttcgtctgaaaccagaatgatgaaggcaatataaatcaaacctattccagcaggtttcatttggtctaatttctctgcagatattaatcattatacagttctatacaaatgacatgtaactccattgtaactcaggatacagaatgttcactctggttctttctctagtgtgctattttgacaatataaaagaaaataaataaattgaaactgtggggcatcaagattgcaagacaccaacaataccaagacattaaagagagaaatggcccatgctaaacctataaaccagcatgcaaattggcaaaaacatttatctgccacagagtcaccataaggaaaaataaactcccttcgtttttcttttgaaaattggtatgtcaggtggaggtgacaaagaattcttcctaaaagttcacagaaagagtattattaattctagtaaagatcatctagaagaccaaggctagtcaaattccatggcatggtatatagtggcagaaaataccagcactcaaattcacagatctacactatagtagatacaaagttgaaggttggaattgtagcaaaggaaaatgtataagaatcaaaatttggttcccattgtgggagctggtgtcaagtaattttacaaaacaccatacatgccttccttttgtctcattgtaacatgttttgtctgacaccaacaaaggatcctcagagaagaatctaaagcccaggaaagcaaaagtaatccagaagcgcaggcagtaatggggcccagaacaagcaacacacctgtgcctatggataaagattcctctgaatctaacaaggctaattgaaaagagaaaaattccatgtcaacatcccttaataaatgtgttcccccaaaatgaattggttggaatagatacaactataaaggaataaagagcaaagggaacgcttattatttgtgcattgttcccccttttattttaattcaccatgcatgcattttcagtaagataactgtgcctataaatacaaaggataacatcagtgcatattttggaagccacttcatttcattattttttgtcagcatttcagtgcaattttttcctagcaggggaaagaaaatcacaataccatatgatctagtagttttacattcctgtcttccccttttcctgctgaatgcagatcagttcatttttgatagtgggtagaaggactttgtaaatatgtttctgacttcagacaacccacatacctttagggaatgatctcccaaagctcactggattttagtatcgcgggatttcccagaaggcaatctaagttggggctctacacatgtgattccccattcattgtatccactcaatactactaacttctttatattagcaatttatggcccttgtcataaccaatgttcgagaagtaaaccatatatattgttttcttcagaattaaacaaaaagttctaaaaactattttaacttcagggaaacatgcccgagtcacagtgactaccagagttactagagcatgtactcttataactcacttacccagaactcatttccagtgttgcaggctacctggacctcacttgataactccactcaaactaggtactttaagcctcctcagagccttttactggccaggtctatgttcatttctatataaacactcacacaaataaatgccatgctgttgtcttagttacttgaatattttaccatgggatgagtgccagtcgagaggtggcccagaataaaaatattgctgttgtgatggttttaaacaggttttctattccagctttgttcactggatgtataaggaatgtcagagcagagaaaactcatgacaggtcaggggtcagaggaacactgccacgaacactccttttgcagtgtttaatttcctgtttaaagaatgtagtagaaatattgggttgactatcatcttaattctttactcttataagggtatctctctatcttgaggccattacagtcaggtctgaaatttaaggaagttggaactttggccattttagttagacccccaaagtctttgacagtacttccagtgacaacacaataatcatttgaccaaagtgagtttcaggatattttccccaaattcaacttcttgacccattaagctctgtgattctttgcaagatcttctgttattaggatgatggtattgccatgtgctatcaagaaacattgaaaagaatcaagacatactggtaagtttacaaacaaagctatgttgtagttaagaccaaatatctgctaatatattaatacagaaaagaataccacttaaattcataaattataattctcttgacaactcaactcccaagataaactttctttttcacttatgtaaaactttcaactccattcaaaccttcaggacaaggaaacattagctgagtctgtcatcctagtgtgaaggcgagaattacaaaaattcagaaagatattcatatactaatcatcactaagaacagaaatcaagacagaacatcttacataataaatgtgcatcaatgaaagatttcaaaaggaagaaattagtcattgttttcctcctacagatatcatccaattgcctttattacctgtgatacacatacacacatgcacacacacgcaataaaacaaattaggagtgcttggcacacaactattaattgacaaattattttttggttaccactgaaatgcatgaggaatgctgaaaataaaactggtcttttaaccttcttgtagcacaagtctatgaaagagctattggtaccttagtaaaatacagagttacatggacggatggctattaacagtttctttttggctgtgtctatacaagtcaggatgtaattgaaaaagatagtttcatttagaaatctgaaaccttaactctggagcttcagttaccttgttgggttgttacagacatcataaaaatgacacagctaaatcctagcatgggcacagccaaagcccgaatcccaaaggcaaacaaaaacggctacaagcaagtaaaaatgtagctttgtagtttaaaatttttataagaaattattaggttgtgtgtggaatacaactttctctaaaacaaacaaaaggccggacccttattcaagtactgtgtgttgtccttagttccacaacaacacaggaacacagaacttaatgtggattatgtggaaaggccacaccattaaactgtgggcagtaagaactctgaaaacatggagaaaagggtgataattcagttcagggtagagaaggctgagtgtggagtcatttagcagaaaattttgtggatatgaatgtttgatttttttaacacaaggaatgtttgaccagctctcctcatcctctcttaatgcagacaaagagcaaagcagtaaaatggagcctgagggtattaatttcacaataaggaatacaatttgttgatgatgagagtcatttgatgttagaaagtgttgtgaagaaaggctgggaaatcttcccaaaagaattttaagaaagagtcagaagctcatccatctgaaatattctaagagagggctgctgggagcaggagcacagcccttgggaggtctaggccctggcatcgtgtgcgtcatgtgtatatacatacttagttgtgcttgtgttgcacaaatactcatgcatacggagtcaatataaactggcacatatagatttgagtgaaaagtcatataaatctgccattccccccaaccccataaacaaaaggaaaaaccaaaattaaaaattccaaacttatgccattgggccagatctttttctaccataccctcattcaaaggagggaggtagaaggatgagagaaaaaacccagtttgggataaatgactcccaaggcctctcagctacttttacgtagctggctctcattatatataagatagttagcacatgggacgaagtaaacaaacaaataactaaaaaagattttcttgtacttccacatctagaaagaaatctaccctgtggatttacatgttaaggtgaactaggtaaagtaggcagtagtatatcaatggactattgtgttctaagaaatgtgcatcattagttgtatttttttcctttaaaatatgaattccttttaggaggttaatttcaaaatgacttttttttttcttttcccgcccccagccctcccttatagatgatacttccttaaaagttcagattgccaaggatgttttctctcaggaaaccgatctggaattttgatttttaggaaatcctggatacatttctccagctcctcctcaattgagagcttttctttaacagctttttttttgctgctcatgttcgattccctggagcctgaagtcagagtccggagtaagtcgcttttccgccgcatctctgactgttggatcagctggacagggcccttcttgatgggacggtccagagtctggatgttggtctggcgtgtcacgggaccacagatgaccgtctcctggggagagctggcctcagactggctgtcgcagctagatgtggagaggtcattgcaagacgtgccgctctccccttctttgtcacctttgccattcttgcagcagcaatcgcagtgtgagggtgaccatctggaaggctcacggtagaagacatattcagtgtagcttgaccagatcttgtcatctgtatattggttgatgaaagatgctgtcaccgatgagttacaggccaccatgtggaatccacactctgacaacatatcaaaagccctttccaggtgcttgaatttgagataaaatctggaggtgtatctttctggggctcgatcagggtctctgctttcattcaaagtttctccaaagacttcttttgccaaggaaatccttccacaaaccaaaatccggggaactctccgaaacttggcatctgcctgtccctctctgcccaaggtgcaggatcctctgtaacccacagtaatgaaaccccacttgcggtcggcagggagcagggaggaaggggggcagattcttgtgtcgcttccttgggaggcatcttcaaagtcactgtggcagaattcatctgggctttgcttgatttcatcgggggtcaggagtttgaccaagtctgggagctggaagtattcagcttcccttttcagtcttcctttttctggaaagtgatcaggcaggaccacctgcctgtccctgagatagtccagaatataacggaacaagaatccatctctgtcaatgaaaaaccttcccttggagtccttggctagatcattagccgtgtctctctttggggaaaacattttccacaggagggaatgagggatgcttatcaatgtggaatggcgagtaaaataaacttgacccccgacattcagctctaccacctcagggaaggagttgggaactgcggacccttgttctcgaggataataacgactacagtttccactcagagccattgtccctttcttctgctgctgctattttgatttaaaggtgcaatccaatggagtcacagccttatcctttggatcaacttgtaagaaagggaaaaggatgctaacttattaaaaaatgacctcctcttatcccagtatttttcccccaagaaatcaaaatgtataagagtccacaggtgaagtgatgctgaaaaagtagtttaaaccctggatggtggatggtagtgagctgctacttcataaaatataatcaactcgtctatatccaatcttccatcaagctcacatgcaaggcaggccaattccccagttactcagatgtccgtctgccggcaagggcaaacggactcccatgttcccagccaggtgggagccggtgcgagccagaggccaacgcagcgcagagatgccggcgg

SEQ ID NO: 19040 - RNA, 6715 nt, Homo sapiens
  source 1..6715: mol_type = other RNA
tggagtccaggaatctgcatttttacaagtgctacacatgatttttgtgcatactgagtattaaaaaacactattaaaaagtttgcaatggagatcactggaaaaagaatctccattccaacgtatacagcaagatgagaataataggcatttcaaacaaataagctctgtgtttgcatcacaaggctgtgattattaaagtttaagactctattctttcagcaggggtagagagcaataaccatttcgtctgaaaccagaatgatgaaggcaatataaatcaaacctattccagcaggtttcatttggtctaatttctctgcagatattaatcattatacagttctatacaaatgacatgtaactccattgtaactcaggatacagaatgttcactctggttctttctctagtgtgctattttgacaatataaaagaaaataaataaattgaaactgtggggcatcaagattgcaagacaccaacaataccaagacattaaagagagaaatggcccatgctaaacctataaaccagcatgcaaattggcaaaaacatttatctgccacagagtcaccataaggaaaaataaactcccttcgtttttcttttgaaaattggtatgtcaggtggaggtgacaaagaattcttcctaaaagttcacagaaagagtattattaattctagtaaagatcatctagaagaccaaggctagtcaaattccatggcatggtatatagtggcagaaaataccagcactcaaattcacagatctacactatagtagatacaaagttgaaggttggaattgtagcaaaggaaaatgtataagaatcaaaatttggttcccattgtgggagctggtgtcaagtaattttacaaaacaccatacatgccttccttttgtctcattgtaacatgttttgtctgacaccaacaaaggatcctcagagaagaatctaaagcccaggaaagcaaaagtaatccagaagcgcaggcagtaatggggcccagaacaagcaacacacctgtgcctatggataaagattcctctgaatctaacaaggctaattgaaaagagaaaaattccatgtcaacatcccttaataaatgtgttcccccaaaatgaattggttggaatagatacaactataaaggaataaagagcaaagggaacgcttattatttgtgcattgttcccccttttattttaattcaccatgcatgcattttcagtaagataactgtgcctataaatacaaaggataacatcagtgcatattttggaagccacttcatttcattattttttgtcagcatttcagtgcaattttttcctagcaggggaaagaaaatcacaataccatatgatctagtagttttacattcctgtcttccccttttcctgctgaatgcagatcagttcatttttgatagtgggtagaaggactttgtaaatatgtttctgacttcagacaacccacatacctttagggaatgatctcccaaagctcactggattttagtatcgcgggatttcccagaaggcaatctaagttggggctctacacatgtgattccccattcattgtatccactcaatactactaacttctttatattagcaatttatggcccttgtcataaccaatgttcgagaagtaaaccatatatattgttttcttcagaattaaacaaaaagttctaaaaactattttaacttcagggaaacatgcccgagtcacagtgactaccagagttactagagcatgtactcttataactcacttacccagaactcatttccagtgttgcaggctacctggacctcacttgataactccactcaaactaggtactttaagcctcctcagagccttttactggccaggtctatgttcatttctatataaacactcacacaaataaatgccatgctgttgtcttagttacttgaatattttaccatgggatgagtgccagtcgagaggtggcccagaataaaaatattgctgttgtgatggttttaaacaggttttctattccagctttgttcactggatgtataaggaatgtcagagcagagaaaactcatgacaggtcaggggtcagaggaacactgccacgaacactccttttgcagtgtttaatttcctgtttaaagaatgtagtagaaatattgggttgactatcatcttaattctttactcttataagggtatctctctatcttgaggccattacagtcaggtctgaaatttaaggaagttggaactttggccattttagttagacccccaaagtctttgacagtacttccagtgacaacacaataatcatttgaccaaagtgagtttcaggatattttccccaaattcaacttcttgacccattaagctctgtgattctttgcaagatcttctgttattaggatgatggtattgccatgtgctatcaagaaacattgaaaagaatcaagacatactggtaagtttacaaacaaagctatgttgtagttaagaccaaatatctgctaatatattaatacagaaaagaataccacttaaattcataaattataattctcttgacaactcaactcccaagataaactttctttttcacttatgtaaaactttcaactccattcaaaccttcaggacaaggaaacattagctgagtctgtcatcctagtgtgaaggcgagaattacaaaaattcagaaagatattcatatactaatcatcactaagaacagaaatcaagacagaacatcttacataataaatgtgcatcaatgaaagatttcaaaaggaagaaattagtcattgttttcctcctacagatatcatccaattgcctttattacctgtgatacacatacacacatgcacacacacgcaataaaacaaattaggagtgcttggcacacaactattaattgacaaattattttttggttaccactgaaatgcatgaggaatgctgaaaataaaactggtcttttaaccttcttgtagcacaagtctatgaaagagctattggtaccttagtaaaatacagagttacatggacggatggctattaacagtttctttttggctgtgtctatacaagtcaggatgtaattgaaaaagatagtttcatttagaaatctgaaaccttaactctggagcttcagttaccttgttgggttgttacagacatcataaaaatgacacagctaaatcctagcatgggcacagccaaagcccgaatcccaaaggcaaacaaaaacggctacaagcaagtaaaaatgtagctttgtagtttaaaatttttataagaaattattaggttgtgtgtggaatacaactttctctaaaacaaacaaaaggccggacccttattcaagtactgtgtgttgtccttagttccacaacaacacaggaacacagaacttaatgtggattatgtggaaaggccacaccattaaactgtgggcagtaagaactctgaaaacatggagaaaagggtgataattcagttcagggtagagaaggctgagtgtggagtcatttagcagaaaattttgtggatatgaatgtttgatttttttaacacaaggaatgtttgaccagctctcctcatcctctcttaatgcagacaaagagcaaagcagtaaaatggagcctgagggtattaatttcacaataaggaatacaatttgttgatgatgagagtcatttgatgttagaaagtgttgtgaagaaaggctgggaaatcttcccaaaagaattttaagaaagagtcagaagctcatccatctgaaatattctaagagagggctgctgggagcaggagcacagcccttgggaggtctaggccctggcatcgtgtgcgtcatgtgtatatacatacttagttgtgcttgtgttgcacaaatactcatgcatacggagtcaatataaactggcacatatagatttgagtgaaaagtcatataaatctgccattccccccaaccccataaacaaaaggaaaaaccaaaattaaaaattccaaacttatgccattgggccagatctttttctaccataccctcattcaaaggagggaggtagaaggatgagagaaaaaacccagtttgggataaatgactcccaaggcctctcagctacttttacgtagctggctctcattatatataagatagttagcacatgggacgaagtaaacaaacaaataactaaaaaagattttcttgtacttccacatctagaaagaaatctaccctgtggatttacatgttaaggtgaactaggtaaagtaggcagtagtatatcaatggactattgtgttctaagaaatgtgcatcattagttgtatttttttcctttaaaatatgaattccttttaggaggttaatttcaaaatgacttttttttttcttttcccgcccccagccctcccttatagatgatacttccttaaaagttcagattgccaaggatgttttctctcaggaaaccgatctggaattttgatttttaggaaatcctggatacatttctccagctcctcctcaattgagagcttttctttaacagctttttttttgctgctcatgttcgattccctggagcctgaagtcagagtccggagtaagtcgcttttccgccgcatctctgactgttggatcagctggacagggcccttcttgatgggacggtccagagtctggatgttggtctggcgtgtcacgggaccacagatgaccgtctcctggggagagctggcctcagactggctgtcgcagctagatgtggagaggtcattgcaagacgtgccgctctccccttctttgtcacctttgccattcttgcagcagcaatcgcagtgtgagggtgaccatctggaaggctcacggtagaagacatattcagtgtagcttgaccagatcttgtcatctgtatattggttgatgaaagatgctgtcaccgatgagttacaggccaccatgtggaatccacactctgacaacatatcaaaagccctttccaggtgcttgaatttgagataaaatctggaggtgtatctttctggggctcgatcagggtctctgctttcattcaaagtttctccaaagacttcttttgccaaggaaatccttccacaaaccaaaatccggggaactctccgaaacttggcatctgcctgtccctctctgcccaaggtgcaggatcctctgtaacccacagtaatgaaaccccacttgcggtcggcagggagcagggaggaaggggggcagattcttgtgtcgcttccttgggaggcatcttcaaagtcactgtggcagaattcatctgggctttgcttgatttcatcgggggtcaggagtttgaccaagtctgggagctggaagtattcagcttcccttttcagtcttcctttttctggaaagtgatcaggcaggaccacctgcctgtccctgagatagtccagaatataacggaacaagaatccatctctgtcaatgaaaaaccttcccttggagtccttggctagatcattagccgtgtctctctttggggaaaacattttccacaggagggaatgagggatgcttatcaatgtggaatggcgagtaaaataaacttgacccccgacattcagctctaccacctcagggaaggagttgggaactgcggacccttgttctcgaggataataacgactacagtttccactcagagccattgtccctttcttctgctgctgctattttgatttaaaggtgcaatccaatggagtcacagccttatcctttggatcaacttgtaagaaagggaaaaggatgctaacttattaaaaaatgacctcctcttatcccagtatttttcccccaagaaatcaaaatgtataagagtccacaggtgaagtgatgctgaaaaagtagtttaaaccctggatggtggatggtagtgagctgctacttcataaaatataatcaactcgtctatatccaatcttccatcaagctcacatgcaaggcaggccaattccccagttactcagatgtccgtcttagtgagtgctggagacccagttcttgtgaaaaaaataataataaccatttgtaaagcaatcaaaatccacagccaaactgagtctggatcttgtcaaatcccaaacaggtaaacgaccgaggtatcaatgaaaagtgccagagaggtgtgctcttggaaaataactattatatatatgcatttatataaatgcctatttgtatttatgtatgtatgtaggtacatatgtgttcattccgtatcttaagttaaaacaagtcgcaaaaaaagttaagccctgatgagaggaggttgggttgaagaagtaaagcagagaaaatattcaaccaaagcttccccaggggaaaagaaaaatggaaaaagaaatctttggaaaggatccttagaagagagttgcaagaggtaccaggacttagaagcttttcagaaagcccagaagcagaaagatggagagatgtgccctgctagggtcccaggtagccaccccacctgccggcaagggcaaacggactcccatgttcccagccaggtgggagccggtgcgagccagaggccaacgcagcgcagagatgccggcggggggcccggggctccggcttctctggcggcggagctgggtggttccacagttcccagtgcagttcggat

SEQ ID NO: 19041 - RNA, 50 nt, Homo sapiens
  source 1..50: mol_type = other RNA
tggagtccaggaatctgcatttttttttttttttttttttttgagataga

SEQ ID NO: 19042 - RNA, 65 nt, Homo sapiens
  source 1..65: mol_type = other RNA
tggagtgtgacaatggtgtttgtgtctaaactatcaaacgccattatcacactaaatagctactg

SEQ ID NO: 19043 - RNA, 2270 nt, Homo sapiens
  source 1..2270: mol_type = other RNA
tggatttttggatcagggattaacacacatgccaacgaaaaggttgaaagttactgtacaaaggaagaaagtggagtctcctgctcccatgtcccacacctgacccctcccacccactagatgcaaaaagctccttcatgcccaagactttcttgtcttcttttctccagctggaaaccaaaagcaagacgcagcaccaggtaaacgactgtagttagggcagaggatggggcaaggggacacccctctcaggtttcatcgtgggccaggaagcatctggtgaaccccaaaatccttcttgagccccacttccccaaccaactactaaacagagaagggccagagggagcgggggccttctcagtccttcatccgtttcccaaattagtcggtgtcctccaacctaataacactgtttctgttcctttcatcatgtcatctgctcagttgggaaaatagttataaaactgtccttcagcttccttatcaaaaggagaaggggccccagcaggggaggagctgtcaccactggaaggatagggggacacgcgcctcctcttagagtctccttcgcccagtcctgaatcactggattccggccggatgggggcaatctcagtccacaccaaggggggaccctggtcctctggtccccgtccctctgagcctccagggccgggttccatgggcagagtccgcatagggcggaaccagctggccgggcccatcttgggagggtactggggtgccacaggccagccagctccaggtgccaggacctcctggcctcggtagtaggacatggtgggcccaggggcagagggcaagaatgcaggcttcatgctgactgctcgaaactcagcctcatagctgtggtcccggggggcccccagccagtaagcctggggaaccacatccttcgcctggccaggaaggtcggggtagaagcggctgggaacaggatactggttgggtaggagaggagagtagtgatctcccccaaggaattgacagttgggtccaggcggggaggggatgctggtgtcaacagatgtgtacatggactcaaagttctcccggaatcctttggcaaaggggttattatcaattttcagctgagtaatctcggcattctggtaggcagtcacggcaatgaactgggtttcttggaaagtaaagatatgcgtgttggaagcgttgcaggctgcctctggctctccgtcgttcacctcaacgatatgcagccggggctggtacttatggagggactggagcacaatcatctgggtcacattgttggacgcccccttgttgtttgtgagctttagtttcccaaatgaaacttcctggcgcatccagtgcgctcctgtgttgggggagtccgggtggacgtacaggcggtttcctggcatgctgccctcggcctttccacactgcacccacttgccgctctggtaccgccagtggtgctggtccaccaagaccacgtccacaaacatcctgtagtggctggtgggctccagcccggccacagtaaatgacaggaatgggaacatccgccgtccctgcttggtgatgatcatctctgtctggtgctgattaaacttggaccacaacaggtggttgttgagcgcgaccctcagtttccccgacacctccagtcccgcgggtagcgcgtagtcctcacgcggccccgggtagagcccggcgcgcgggtccggggcggcgtagccctcgcccggctggtagccctcggcgtccgcgggcggcgggaaggactcgcccgcgccggggaagccggccgcctggggtcgcggcgggtaggcgtaggctccaaggaagcggctcggcggggcgggcaccaaggcgccccccgggtagggagaccccaggctgccgcccccgcgacgctcgtccgcgtcctgcgcgcccggctccgggtagaagtagcggtgctgcgggtcggcgccaggcgcccggccctcgtcgctccccggcatcggctcggtgcccgtcagcatgtctccgcaacccggctccacgatgcccatccggggcgggctggcaccttcccgtagccgtcgaggacccgcccctccgcgcgcgagagggtcgcgtgggctgggatgggcagggagcagggggcgggggacccgagggccgggtgggggaccccaccggagcccgggctctgacgcctggcttctacgccctcgtccggcaggcgcgcggcagctctcgggcttcctctccagcgggccgctgtcact

SEQ ID NO: 19044 - RNA, 3085 nt, Homo sapiens
  source 1..3085: mol_type = other RNA
tggcagggaggctgggaggggatgggaggagtggagtgggcagccccccacttccaccccgcagcagctcagacgccagctcagaaccggttcttaccaccggcagattgagagtctgtgtcgggggagggggcatcaagtaactgctggaggaagaccccagtccgcagtctatggaaactggtcctgcggcggtcccgggagagcgtccgatggggctgcgagtcagggaggaggatgcagggcgtcaagggacaggcgaaggactggcaggaggggaaactgggaggccagcaggtggaagagacgctgaggtaggggcaaggcagggctgagagccgggtctcgcagcaggaggtgccgggccctggggaactaggcaggccaggaggagcagtgaagagccgagagtccggctcgatcggtgcgggctgctgggccccccgatccttgggtcccaaccttggaaagacctgacgcccccaaagcccgttcctagagccggacccccacacccccattccatcttctgggacagggcacacccggaaggcgagggcagtccggctggcactgggggaaaagaatttttcccagggattcggcagcgggctcttcctcctgcagaaagtcgttttcttcttaatctccttggcccagcccctccagcgaagcctcctggcgcccgagcgtccgaggcgggtgcccggggctgggccgcgctgcggtccgcgctgattgtgtgtcacagaaacatccggcgcgcgccagcaggtcgcgcccgagtccggcagggtggctggcgggcttcggggctggcttggtggaggccgggacgagctgggccgaatccccctcacggcgccgcgcagtccaggcaggcggggaggggcggcaggcggggctgggggcggcgggcccgggcctgagggtcccgcccacggctccacccgtcctgtccgaccttcgaggggggtgatgtgaagggttgcgggggtcgtgggatggggtgaggctggggcggtggccgggaggcatcgcgtcgcgtcggtcctccctccctccggggtggggtcagacggggacgatgtggaggccgaagctgtcggcctgaagcttgatgtggtccccgcggtaactagtggcggtcataggcagcggcagcagcggcaggggcggagccccggggggcggcactataataataaggggaacttagtaaggcggggttgctgaatctccaagcctcgttgtaggccgtgtactgggggtggctgtacgggttgccggagaactcgctccagtgggttgcacacaagggggcacttctgcaagcttcctccccggcttgctcatgagggaggatgagggaccaactgcagcctcaggcaccattcctgccagggtggaggtggggtagcttccctggccagtggggggcacgtgaggggggtaaccaggcagagtggtgctcgccatgtcacgaccagtcacaactgggtatgtctgtgtgcctgacacgttgctgcccagctcagggttggtggatgcagatagactcgacttgacttcatcaagcccaggggtcagggctgggagggagtactcgttcccctgttctgatttgatgtgctctgatgcctggaagacgtcagggtaggaaggacgctcaaagacccgatccaaagcttccagctgctgctgggtgaaggtgtcagctcgcaagtgcttccgcaaactgtccacaccactctgggaatctccattggggactgagccctcagacacatcttcatcacgtttcctcttctcaccattggagcgaggaatccccaggatcccattgatggagtaggatcccactgggtcattggaggcgctggaaacaggaggggaggccgtgctgggaacaatggtgtggccaggggcggtcactcctgtcccagccccatccggcgttgggtggaaaggctgctgaactttggtccggatgattctgttgatggaagagacgctgggcactgtgtcattgtcacagatgccctcggccaggagccggtctcgaatctcccaggcgaacatagtcgggttctgtcgtttgtattcagcaatcttgtccaccactttgggcgtcgccactttgggcttggagccaccgatcacacccggcttgatgctgccggtctcgtagtacctgcccaggattttgctgacacagccgtggctgacccgcagctgccgggagatgtcacagggccgcacaccctggtgggccagctccacgatgcgctgcctcaccacgtcgggtaggggccggccgttcacaaacacccccccgagctggttcacacccccgtgccctgggtgcatcgcggagaaggggtctgctttgcagtgcatatccatggggaggcagaggagcgggagcagcgcggccgccgccgccgtgtcgcctctcaaactcaacttcaggacttgaggagaaaagggagggacggtgggggagggaggatgagtgaacgcccggctgctgcggggcgcgcgggggcggggggcgcagcactgcgctccccgctggggctcctccgggttggccggagcttgcaactgcagtagccgcaacttgccactgtcggggctcggggctgggcggtcagcagaatggccccggggcggtgggccgggccggggtgcactgggggcgcatggctcgcgctgcagctgcagccagggctgaagctgggcgggggaggcgactcgctcagctcccctggaacctggtcatccgagaggcggtggtcggagagcgcgcggggcgggggcggtcagagggcgccgggaggggagccgggcctctccaagtgctggcgagttggcgaagttggcagagaagtagcaatcccggggatgtccgaggtggcgcctgcgggaggggagcgcgcgggccaggcccccgcccccggaaaaggcaggcgcacgccgccgcggccgaagggccgggagggagggagggagccgagcggcgctggcagctctgggctggccccaggtgggttgcggctgcgagaagactcggccggagact

SEQ ID NO: 19045 - RNA, 3071 nt, Homo sapiens
  source 1..3071: mol_type = other RNA
tggcagggaggctgggaggggatgggaggagtggagtgggcagccccccacttccaccccgcagcagctcagacgccagctcagaaccggttcttaccaccggcagattgagagtctgtgtcgggggagggggcatcaagtaactgctggaggaagaccccagtccgcagtctatggaaactggtcctgcggcggtcccgggagagcgtccgatggggctgcgagtcagggaggaggatgcagggcgtcaagggacaggcgaaggactggcaggaggggaaactgggaggccagcaggtggaagagacgctgaggtaggggcaaggcagggctgagagccgggtctcgcagcaggaggtgccgggccctggggaactaggcaggccaggaggagcagtgaagagccgagagtccggctcgatcggtgcgggctgctgggccccccgatccttgggtcccaaccttggaaagacctgacgcccccaaagcccgttcctagagccggacccccacacccccattccatcttctgggacagggcacacccggaaggcgagggcagtccggctggcactgggggaaaagaatttttcccagggattcggcagcgggctcttcctcctgcagaaagtcgttttcttcttaatctccttggcccagcccctccagcgaagcctcctggcgcccgagcgtccgaggcgggtgcccggggctgggccgcgctgcggtccgcgctgattgtgtgtcacagaaacatccggcgcgcgccagcaggtcgcgcccgagtccggcagggtggctggcgggcttcggggctggcttggtggaggccgggacgagctgggccgaatccccctcacggcgccgcgcagtccaggcaggcggggaggggcggcaggcggggctgggggcggcgggcccgggcctgagggtcccgcccacggctccacccgtcctgtccgaccttcgaggggggtgatgtgaagggttgcgggggtcgtgggatggggtgaggctggggcggtggccgggaggcatcgcgtcgcgtcggtcctccctccctccggggtggggtcagacggggacgatgtggaggccgaagctgtcggcctgaagcttgatgtggtccccgcggtaactagtggcggtcataggcagcggcagcagcggcaggggcggagccccggggggcggcactataataataaggggaacttagtaaggcggggttgctgaatctccaagcctcgttgtaggccgtgtactgggggtggctgtacgggttgccggagaactcgctcccaggcaccattcctgccagggtggaggtggggtagcttccctggccagtggggggcacgtgaggggggtaaccaggcagagtggtgctcgccatgtcacgaccagtcacaactgggtatgtctgtgtgcctgacacgttgctgcccagctcagggttggtggatgcagatagactcgacttgacttcatcaagcccaggggtcagggctgggagggagtactcgttcccctgttctgatttgatgtgctctgatgcctggaagacgtcagggtaggaaggacgctcaaagacccgatccaaagcttccagctgctgctgggtgaaggtgtcagctcgcaagtgcttccgcaaactgtccacaccactctgggaatctccattggggactgagccctcagacacatctcttaaagtccagaccagatgcaaacctccacctcctctaatgtgggcaggatcagtgtatacctcaacttcatcacgtttcctcttctcaccattggagcgaggaatccccaggatcccattgatggagtaggatcccactgggtcattggaggcgctggaaacaggaggggaggccgtgctgggaacaatggtgtggccaggggcggtcactcctgtcccagccccatccggcgttgggtggaaaggctgctgaactttggtccggatgattctgttgatggaagagacgctgggcactgtgtcattgtcacagatgccctcggccaggagccggtctcgaatctcccaggcgaacatagtcgggttctgtcgtttgtattcagcaatcttgtccaccactttgggcgtcgccactttgggcttggagccaccgatcacacccggcttgatgctgccggtctcgtagtacctgcccaggattttgctgacacagccgtggctgacccgcagctgccgggagatgtcacagggccgcacaccctggtgggccagctccacgatgcgctgcctcaccacgtcgggtaggggccggccgttcacaaacacccccccgagctggttcacacccccgtgccctgggtgcatcgcggagaaggggtctgctttgcagtgcatatccatggggaggcagaggagcgggagcagcgcggccgccgccgccgtgtcgcctctcaaactcaacttcaggacttgaggagaaaagggagggacggtgggggagggaggatgagtgaacgcccggctgctgcggggcgcgcgggggcggggggcgcagcactgcgctccccgctggggctcctccgggttggccggagcttgcaactgcagtagccgcaacttgccactgtcggggctcggggctgggcggtcagcagaatggccccggggcggtgggccgggccggggtgcactgggggcgcatggctcgcgctgcagctgcagccagggctgaagctgggcgggggaggcgactcgctcagctcccctggaacctggtcatccgagaggcggtggtcggagagcgcgcggggcgggggcggtcagagggcgccgggaggggagccgggcctctccaagtgctggcgagttggcgaagttggcagagaagtagcaatcccggggatgtccgaggtggcgcctgcgggaggggagcgcgcgggccaggcccccgcccccggaaaaggcaggcgcacgccgccgcggccgaagggccgggagggagggagggagccgagcggcgctggcagctctgggctggccccaggtgggttgcggctgcgagaagactcggccggagact

SEQ ID NO: 19046 - RNA, 2729 nt, Homo sapiens
  source 1..2729: mol_type = other RNA
tggcagggaggctgggaggggatgggaggagtggagtgggcagccccccacttccaccccgcagcagctcagacgccagctcagaaccggttcttaccaccggcagattgagagtctgtgtcgggggagggggcatcaagtaactgctggaggaagaccccagtccgcagtctatggaaactggtcctgcggcggtcccgggagagcgtccgatggggctgcgagtcagggaggaggatgcagggcgtcaagggacaggcgaaggactggcaggaggggaaactgggaggccagcaggtggaagagacgctgaggtaggggcaaggcagggctgagagccgggtctcgcagcaggaggtgccgggccctggggaactaggcaggccaggaggagcagtgaagagccgagagtccggctcgatcggtgcgggctgctgggccccccgatccttgggtcccaaccttggaaagacctgacgcccccaaagcccgttcctagagccggacccccacacccccattccatcttctgggacagggcacacccggaaggcgagggcagtccggctggcactgggggaaaagaatttttcccagggattcggcagcgggctcttcctcctgcagaaagtcgttttcttcttaatctccttggcccagcccctccagcgaagcctcctggcgcccgagcgtccgaggcgggtgcccggggctgggccgcgctgcggtccgcgctgattgtgtgtcacagaaacatccggcgcgcgccagcaggtcgcgcccgagtccggcagggtggctggcgggcttcggggctggcttggtggaggccgggacgagctgggccgaatccccctcacggcgccgcgcagtccaggcaggcggggaggggcggcaggcggggctgggggcggcgggcccgggcctgagggtcccgcccacggctccacccgtcctgtccgaccttcgaggggggtgatgtgaagggttgcgggggtcgtgggatggggtgaggctggggcggtggccgggaggcatcgcgtcgcgtcggtcctccctccctccggggtggggtcagacggggacgatgtggaggccgaagctgtcggcctgaagcttgatgtggtccccgcggtaactagtggcggtcataggcagcggcagcagcggcaggggcggagccccggggggcggcactataataataaggggaacttagtaaggcggggttgctgaatctccaagcctcgttgtaggccgtgtactgggggtggctgtacgggttgccggagaactcgctcccaggcaccattcctgccagggtggaggtggggtagcttccctggccagtggggggcacgtgaggggggtaaccaggcagagtggtgctcgccatgtcacgaccagtcacaactgggtatgtctgtgtgcctgacacgttgctgcccagctcagggttggtggatgcagatagactcgacttgacttcatcaagcccaggggtcagggctgggagggagtactcgttcccctgttctgatttgatgtgctctgatgcctggaagacgtcagggtaggaaggacgctcaaagacccgatccaaagcttccagctgctgctgggtgaaggtgtcagctcgcaagtgcttccgcaaactgtccacaccactctgggaatctccattggggactgagccctcagacacatcttcatcacgtttcctcttctcaccattggagcgaggaatccccaggatcccattgatggagtaggatcccactgggtcattggaggcgctggaaacaggaggggaggccgtgctgggaacaatggtgtggccaggggcggtcactcctgtcccagccccatccggcgttgggtggaaaggctgctgaactttggtccggatgattctgttgatggaagagacgctgggcactgtgtcattgtcacagatgccctcggccaggagccggtctcgaatctcccaggcgaacatagtcgggttctgtcgtttgtattcagcaatcttgtccaccactttgggcgtcgccactttgggcttggagccaccgatcacacccggcttgatgctgccggtctcgtagtacctgcccaggattttgctgacacagccgtggctgacccgcagctgccgggagatgtcacagggccgcacaccctggtgggccagctccacgatgcgctgcctcaccacgtcgggtaggggccggccgttcacaaacacccccccgagctggttcacacccccgtgccctgggtgcatcgcggagaaggggtctgctttgcagtgcatatccatggggaggcagaggagcgggagcagcgcggccgccgccgccgtgtcgcctctcaaactcaacttcaggactgccggacccgcgcgctcttccatgctaggctccccgcggccgccgcgtcctggggctgggtctggctgtcccgctcctccgcggcccgacaacgcgtctcgccttcgccgccgccgccgcccggagatctgggcgcagccacccaacaccaagcggctcagataacccgagccgcccgccgccacggctgtgtgctccgcccgcgcccgctctctcactcccggccgcgcagaggctccggcaccccgaggagcccgggttctccgccccgcgcacacgcgtgcacacgcaccgaggccccagccagccgcaggcaagcagccaccctcgctgcct

SEQ ID NO: 19047 - RNA, 3002 nt, Homo sapiens
  source 1..3002: mol_type = other RNA
tggcagggaggctgggaggggatgggaggagtggagtgggcagccccccacttccaccccgcagcagctcagacgccagctcagaaccggttcttaccaccggcagattgagagtctgtgtcgggggagggggcatcaagtaactgctggaggaagaccccagtccgcagtctatggaaactggtcctgcggcggtcccgggagagcgtccgatggggctgcgagtcagggaggaggatgcagggcgtcaagggacaggcgaaggactggcaggaggggaaactgggaggccagcaggtggaagagacgctgaggtaggggcaaggcagggctgagagccgggtctcgcagcaggaggtgccgggccctggggaactaggcaggccaggaggagcagtgaagagccgagagtccggctcgatcggtgcgggctgctgggccccccgatccttgggtcccaaccttggaaagacctgacgcccccaaagcccgttcctagagccggacccccacacccccattccatcttctgggacagggcacacccggaaggcgagggcagtccggctggcactgggggaaaagaatttttcccagggattcggcagcgggctcttcctcctgcagaaagtcgttttcttcttaatctccttggcccagcccctccagcgaagcctcctggcgcccgagcgtccgaggcgggtgcccggggctgggccgcgctgcggtccgcgctgattgtgtgtcacagaaacatccggcgcgcgccagcaggtcgcgcccgagtccggcagggtggctggcgggcttcggggctggcttggtggaggccgggacgagctgggccgaatccccctcacggcgccgcgcagtccaggcaggcggggaggggcggcaggcggggctgggggcggcgggcccgggcctgagggtcccgcccacggctccacccgtcctgtccgaccttcgaggggggtgatgtgaagggttgcgggggtcgtgggatggggtgaggctggggcggtggccgggaggcatcgcgtcgcgtcggtcctccctccctccggggtggggtcagacggggacgatgtggaggccgaagctgtcggcctgaagcttgatgtggtccccgcggtaactagtggcggtcataggcagcggcagcagcggcaggggcggagccccggggggcggcactataataataaggggaacttagtaaggcggggttgctgaatctccaagcctcgttgtaggccgtgtactgggggtggctgtacgggttgccggagaactcgctcccaggcaccattcctgccagggtggaggtggggtagcttccctggccagtggggggcacgtgaggggggtaaccaggcagagtggtgctcgccatgtcacgaccagtcacaactgggtatgtctgtgtgcctgacacgttgctgcccagctcagggttggtggatgcagatagactcgacttgacttcatcaagcccaggggtcagggctgggagggagtactcgttcccctgttctgatttgatgtgctctgatgcctggaagacgtcagggtaggaaggacgctcaaagacccgatccaaagcttccagctgctgctgggtgaaggtgtcagctcgcaagtgcttccgcaaactgtccacaccactctgggaatctccattggggactgagccctcagacacatcttcatcacgtttcctcttctcaccattggagcgaggaatccccaggatcccattgatggagtaggatcccactgggtcattggaggcgctggaaacaggaggggaggccgtgctgggaacaatggtgtggccaggggcggtcactcctgtcccagccccatccggcgttgggtggaaaggctgctgaactttggtccggatgattctgttgatggaagagacgctgggcactgtgtcattgtcacagatgccctcggccaggagccggtctcgaatctcccaggcgaacatagtcgggttctgtcgtttgtattcagcaatcttgtccaccactttgggcgtcgccactttgggcttggagccaccgatcacacccggcttgatgctgccggtctcgtagtacctgcccaggattttgctgacacagccgtggctgacccgcagctgccgggagatgtcacagggccgcacaccctggtgggccagctccacgatgcgctgcctcaccacgtcgggtaggggccggccgttcacaaacacccccccgagctggttcacacccccgtgccctgggtgcatcgcggagaaggggtctgctttgcagtgcatatccatggggaggcagaggagcgggagcagcgcggccgccgccgccgtgtcgcctctcaaactcaacttcaggacttgaggagaaaagggagggacggtgggggagggaggatgagtgaacgcccggctgctgcggggcgcgcgggggcggggggcgcagcactgcgctccccgctggggctcctccgggttggccggagcttgcaactgcagtagccgcaacttgccactgtcggggctcggggctgggcggtcagcagaatggccccggggcggtgggccgggccggggtgcactgggggcgcatggctcgcgctgcagctgcagccagggctgaagctgggcgggggaggcgactcgctcagctcccctggaacctggtcatccgagaggcggtggtcggagagcgcgcggggcgggggcggtcagagggcgccgggaggggagccgggcctctccaagtgctggcgagttggcgaagttggcagagaagtagcaatcccggggatgtccgaggtggcgcctgcgggaggggagcgcgcgggccaggcccccgcccccggaaaaggcaggcgcacgccgccgcggccgaagggccgggagggagggagggagccgagcggcgctggcagctctgggctggccccaggtgggttgcggctgcgagaagactcggccggagact

SEQ ID NO: 19048 - RNA, 3052 nt, Homo sapiens
  source 1..3052: mol_type = other RNA
tggcagggaggctgggaggggatgggaggagtggagtgggcagccccccacttccaccccgcagcagctcagacgccagctcagaaccggttcttaccaccggcagattgagagtctgtgtcgggggagggggcatcaagtaactgctggaggaagaccccagtccgcagtctatggaaactggtcctgcggcggtcccgggagagcgtccgatggggctgcgagtcagggaggaggatgcagggcgtcaagggacaggcgaaggactggcaggaggggaaactgggaggccagcaggtggaagagacgctgaggtaggggcaaggcagggctgagagccgggtctcgcagcaggaggtgccgggccctggggaactaggcaggccaggaggagcagtgaagagccgagagtccggctcgatcggtgcgggctgctgggccccccgatccttgggtcccaaccttggaaagacctgacgcccccaaagcccgttcctagagccggacccccacacccccattccatcttctgggacagggcacacccggaaggcgagggcagtccggctggcactgggggaaaagaatttttcccagggattcggcagcgggctcttcctcctgcagaaagtcgttttcttcttaatctccttggcccagcccctccagcgaagcctcctggcgcccgagcgtccgaggcgggtgcccggggctgggccgcgctgcggtccgcgctgattgtgtgtcacagaaacatccggcgcgcgccagcaggtcgcgcccgagtccggcagggtggctggcgggcttcggggctggcttggtggaggccgggacgagctgggccgaatccccctcacggcgccgcgcagtccaggcaggcggggaggggcggcaggcggggctgggggcggcgggcccgggcctgagggtcccgcccacggctccacccgtcctgtccgaccttcgaggggggtgatgtgaagggttgcgggggtcgtgggatggggtgaggctggggcggtggccgggaggcatcgcgtcgcgtcggtcctccctccctccggggtggggtcagacggggacgatgtggaggccgaagctgtcggcctgaagcttgatgtggtccccgcggtaactagtggcggtcataggcagcggcagcagcggcaggggcggagccccggggggcggcattagtaaggcggggttgctgaatctccaagcctcgttgtaggccgtgtactgggggtggctgtacgggttgccggagaactcgctcccaggcaccattcctgccagggtggaggtggggtagcttccctggccagtggggggcacgtgaggggggtaaccaggcagagtggtgctcgccatgtcacgaccagtcacaactgggtatgtctgtgtgcctgacacgttgctgcccagctcagggttggtggatgcagatagactcgacttgacttcatcaagcccaggggtcagggctgggagggagtactcgttcccctgttctgatttgatgtgctctgatgcctggaagacgtcagggtaggaaggacgctcaaagacccgatccaaagcttccagctgctgctgggtgaaggtgtcagctcgcaagtgcttccgcaaactgtccacaccactctgggaatctccattggggactgagccctcagacacatctcttaaagtccagaccagatgcaaacctccacctcctctaatgtgggcaggatcagtgtatacctcaacttcatcacgtttcctcttctcaccattggagcgaggaatccccaggatcccattgatggagtaggatcccactgggtcattggaggcgctggaaacaggaggggaggccgtgctgggaacaatggtgtggccaggggcggtcactcctgtcccagccccatccggcgttgggtggaaaggctgctgaactttggtccggatgattctgttgatggaagagacgctgggcactgtgtcattgtcacagatgccctcggccaggagccggtctcgaatctcccaggcgaacatagtcgggttctgtcgtttgtattcagcaatcttgtccaccactttgggcgtcgccactttgggcttggagccaccgatcacacccggcttgatgctgccggtctcgtagtacctgcccaggattttgctgacacagccgtggctgacccgcagctgccgggagatgtcacagggccgcacaccctggtgggccagctccacgatgcgctgcctcaccacgtcgggtaggggccggccgttcacaaacacccccccgagctggttcacacccccgtgccctgggtgcatcgcggagaaggggtctgctttgcagtgcatatccatggggaggcagaggagcgggagcagcgcggccgccgccgccgtgtcgcctctcaaactcaacttcaggacttgaggagaaaagggagggacggtgggggagggaggatgagtgaacgcccggctgctgcggggcgcgcgggggcggggggcgcagcactgcgctccccgctggggctcctccgggttggccggagcttgcaactgcagtagccgcaacttgccactgtcggggctcggggctgggcggtcagcagaatggccccggggcggtgggccgggccggggtgcactgggggcgcatggctcgcgctgcagctgcagccagggctgaagctgggcgggggaggcgactcgctcagctcccctggaacctggtcatccgagaggcggtggtcggagagcgcgcggggcgggggcggtcagagggcgccgggaggggagccgggcctctccaagtgctggcgagttggcgaagttggcagagaagtagcaatcccggggatgtccgaggtggcgcctgcgggaggggagcgcgcgggccaggcccccgcccccggaaaaggcaggcgcacgccgccgcggccgaagggccgggagggagggagggagccgagcggcgctggcagctctgggctggccccaggtgggttgcggctgcgagaagactcggccggagact

SEQ ID NO: 19049 - RNA, 2983 nt, Homo sapiens
  source 1..2983: mol_type = other RNA
tggcagggaggctgggaggggatgggaggagtggagtgggcagccccccacttccaccccgcagcagctcagacgccagctcagaaccggttcttaccaccggcagattgagagtctgtgtcgggggagggggcatcaagtaactgctggaggaagaccccagtccgcagtctatggaaactggtcctgcggcggtcccgggagagcgtccgatggggctgcgagtcagggaggaggatgcagggcgtcaagggacaggcgaaggactggcaggaggggaaactgggaggccagcaggtggaagagacgctgaggtaggggcaaggcagggctgagagccgggtctcgcagcaggaggtgccgggccctggggaactaggcaggccaggaggagcagtgaagagccgagagtccggctcgatcggtgcgggctgctgggccccccgatccttgggtcccaaccttggaaagacctgacgcccccaaagcccgttcctagagccggacccccacacccccattccatcttctgggacagggcacacccggaaggcgagggcagtccggctggcactgggggaaaagaatttttcccagggattcggcagcgggctcttcctcctgcagaaagtcgttttcttcttaatctccttggcccagcccctccagcgaagcctcctggcgcccgagcgtccgaggcgggtgcccggggctgggccgcgctgcggtccgcgctgattgtgtgtcacagaaacatccggcgcgcgccagcaggtcgcgcccgagtccggcagggtggctggcgggcttcggggctggcttggtggaggccgggacgagctgggccgaatccccctcacggcgccgcgcagtccaggcaggcggggaggggcggcaggcggggctgggggcggcgggcccgggcctgagggtcccgcccacggctccacccgtcctgtccgaccttcgaggggggtgatgtgaagggttgcgggggtcgtgggatggggtgaggctggggcggtggccgggaggcatcgcgtcgcgtcggtcctccctccctccggggtggggtcagacggggacgatgtggaggccgaagctgtcggcctgaagcttgatgtggtccccgcggtaactagtggcggtcataggcagcggcagcagcggcaggggcggagccccggggggcggcattagtaaggcggggttgctgaatctccaagcctcgttgtaggccgtgtactgggggtggctgtacgggttgccggagaactcgctcccaggcaccattcctgccagggtggaggtggggtagcttccctggccagtggggggcacgtgaggggggtaaccaggcagagtggtgctcgccatgtcacgaccagtcacaactgggtatgtctgtgtgcctgacacgttgctgcccagctcagggttggtggatgcagatagactcgacttgacttcatcaagcccaggggtcagggctgggagggagtactcgttcccctgttctgatttgatgtgctctgatgcctggaagacgtcagggtaggaaggacgctcaaagacccgatccaaagcttccagctgctgctgggtgaaggtgtcagctcgcaagtgcttccgcaaactgtccacaccactctgggaatctccattggggactgagccctcagacacatcttcatcacgtttcctcttctcaccattggagcgaggaatccccaggatcccattgatggagtaggatcccactgggtcattggaggcgctggaaacaggaggggaggccgtgctgggaacaatggtgtggccaggggcggtcactcctgtcccagccccatccggcgttgggtggaaaggctgctgaactttggtccggatgattctgttgatggaagagacgctgggcactgtgtcattgtcacagatgccctcggccaggagccggtctcgaatctcccaggcgaacatagtcgggttctgtcgtttgtattcagcaatcttgtccaccactttgggcgtcgccactttgggcttggagccaccgatcacacccggcttgatgctgccggtctcgtagtacctgcccaggattttgctgacacagccgtggctgacccgcagctgccgggagatgtcacagggccgcacaccctggtgggccagctccacgatgcgctgcctcaccacgtcgggtaggggccggccgttcacaaacacccccccgagctggttcacacccccgtgccctgggtgcatcgcggagaaggggtctgctttgcagtgcatatccatggggaggcagaggagcgggagcagcgcggccgccgccgccgtgtcgcctctcaaactcaacttcaggacttgaggagaaaagggagggacggtgggggagggaggatgagtgaacgcccggctgctgcggggcgcgcgggggcggggggcgcagcactgcgctccccgctggggctcctccgggttggccggagcttgcaactgcagtagccgcaacttgccactgtcggggctcggggctgggcggtcagcagaatggccccggggcggtgggccgggccggggtgcactgggggcgcatggctcgcgctgcagctgcagccagggctgaagctgggcgggggaggcgactcgctcagctcccctggaacctggtcatccgagaggcggtggtcggagagcgcgcggggcgggggcggtcagagggcgccgggaggggagccgggcctctccaagtgctggcgagttggcgaagttggcagagaagtagcaatcccggggatgtccgaggtggcgcctgcgggaggggagcgcgcgggccaggcccccgcccccggaaaaggcaggcgcacgccgccgcggccgaagggccgggagggagggagggagccgagcggcgctggcagctctgggctggccccaggtgggttgcggctgcgagaagactcggccggagact

SEQ ID NO: 19050 - RNA, 4617 nt, Homo sapiens
  source 1..4617: mol_type = other RNA
tggcagggaggctgggaggggcactgcctcccacaaggagctcacgttctggtgggaggaggccaagaatcaggaccaaggagaacttcagtgaagcaaaagaagaaaaatggaacaggggtgaaggggctggagaagcctcagggaggtgacagctgaaacctgcaccaggaggggcggggcctgtagtgggcactgggcagtaggaccctgtggtgagccaggtctgctcaggtaacaggaaggtcgttgggccacagtgtggtggggactgccctgaggccgggtggctgcagctgggcctggtgtgggggtggtggccttgcctgggggcccctgcagggctggcctagcagggaaggtgtccacaccatctcagctctgggcaggtggggtggacctggggcttatccaccgtctagaaaccacttggaggccaggcagccttggctactgctctgtggctgggcctccagggccctcctggtcatgcagaatggggcagagccggagcccgttgggagggagcctgggctgtgcgctcggggtactgtgaagtccctggaggcctggacccccatcctttcctgggtgggtcagggacagggtgggacagggacagagggcaagggtgagagggtagagagcgggcaacaggtagtaacagccggcccttctctcccagcacagcgactcggactccgaccccgagtactccacgctgccgccatccatccccagtgcggtgcccgtgaccggcgagtccttctgtgactgtgctgggcagagcgaggcctccttctgtagcagcctgcactcggcccaccggggcagggactgccgctgcggagaggaagacgagtgtgagcgtggggcccagcccctgctgggactgcactgcgggcgggcctgggggtgggcagggcagagccccatggagctctcagggctgccccagcctgggcctctcttgcagatttcgactgggtctgggatgacttaaataagtcatcagccaccctgctgagctgtgacaaccgtaaggtcagcttccacatggagtacagctgcggcacagcggccatccggggcaccaaggagctgggggagggccagcacttctgggagatcaagatgacctctcccgtctacggcaccgacatggtaagttgcttcggcccagggtgcttctggggaacctggctccggcagcccagccccgcgccctctgcctggcccctgttcctagatggtgggcatcgggacgtcggatgtggacctggacaaataccgccacacgttctgcagcctgctgggcagggatgaggacagctggggcctctcctacacgggtgcgtgaggcccagggtggggcggggccgagcctggagctcccgggctcactgcgaccctggctgcccccaggcctcctccaccacaagggcgacaagaccagcttctcatcgcggttcggccagggctccatcattggcgtgcacctggacacctggcacggcacactcacctttttcaagaacaggaagtgtataggtgaggccgtcacaggacttgagctcctctcagctgtcaccccgagggaggcagccaccccgccccagcccaggggacactgaggttttctgaaagggttcctcccagaagcctgaggccccagggtcccagggggtgggacagtgaggccaggctggagtggcagggccagcgcgtgcaccctgccttgcctcagctgtgccagctgcccacccgggtgactgtagcgtgaggtctgaggggctgcgcccagtagctggccccttccctgcctggggttcaggctgggcccctcccttccaggtgtggcagccaccaagctgcagaacaagagattctacccgatggtgtgctccacggcggcccggagcagcatgaaggtcacccgctcctgtgccagcgccacttccctccagtacctgtgctgccaccgcctgcgccagctgcggccagactcgggagacacgctggagggtctgccgctgccgccgggcctcaagcaggtgctacacaacaagctgggctgggtcctgagcatgagttgcagccgccgcaaggctccagtgtccgatccccaggcagcgacctccgcccaccccagcagtcgcgagcctcggccctgccagaggaagcgctgccgccggacctgactgacttcccagtggaactgccttcttgggctgggacagcccctttcctctgtcccttctttctctgtcccttccttccagccacactccagggcggagttggatgaggcccgtccggagggagccatctcttgctcccgaggctgggacagtcctttctgtgggggctctagggcccctctgctgctgtgctgggtggggaagcggctgccctgagccccaggtcttgtgggaggctgcgaggacgagagcctggctggagcccgcgttgctgttcccacagggcctcggtttttcctaacttgctctgcatgctgtcagcggctgccccgccgtcatagacttaaaggactgcaataaatgtagagttgatgtctaacacccacatggcgtgagctgaaacgtatccgtgcagaggccgggcttgcgagcagcctgggccttctcccaggcctcactgcccctccacatccttgggagtcccctactgcttctggctgagggtgccacaccccaagcctccaggtggcagtggggccctggagctgccttctggtccctgccgagtgtgtgtgtgtgttgggggggcacagccctgctgctgaggcctcccctggggcctacgtgttcaggactcagcacaggaaccgccagccatctgccagccagaagcccctcttctcccagctacctaaaacttcccctgcaaccacccacccttcccctgaggtcagacctgctcagccagagaacccacccaggctgagggtccacatgtggctgggggtcctcccccaccgcccagggtgtctggtctgtccccaaggctgcatgctgtcctggtggtcccacgtgtggtcaggagcccaggtccagcaggagatcagggttggctgtggtcaggaagaggcagatgcggcgggagaggtcaggccccaccctgcggggacgcccgccttcactgggcggcacaggaaggtcggccaggaggcccatgcgctcccgctccgtgctgcaggcctccagcgcctgctgcagaaggcggggggaggggaaggctgtgacaactgcatcagccacggctgggctgacccgactgaactgcctgatctgcctccgccaggccgcctgcagccctgcgccgtctcttgccactggctcgccggctgcccagcgccctgctgtgcagaaggagaaggcctgggattcccggtactgcttgaggggatactgggcgagagccttggtaacggcgcacacgtgccgactcagctcctgccaagaggccaccagtagcacgtccaggtttgcccagagctgcaggagtaccagggcctcttccacctccggccagctgacggccacctcggcaccggccaccttcgggctctctggctgctgtgtcccccgggaaacgtgctggcgagaccacaggtaggcatccagcccgatgacagccaggtggggccgggcggtggtctcgggggagatccagggcacccagtgggttgggccagagatctgggtcagtgtggcgacgccctgcagaaactcctcgggctccagcagcagcagcaattcctgttcacctgcagcccacacttcaggaggcaggctgcgggggcaggggtcgggactcgctcgggtccaccgcaggctgcgggccgggcgctggggctcgatgcggcactcgcagcccagggcctccagggcctccatcaggacgtcggcaccggcgtcttccaggatggctgtgtccacgcacaccgcgaggcgcttcaggacctgctccggccgcagcagccgcaacgcctcggcagccgccctgcgctcacccgctgggtcccgggctctcgcggcggcctccgagccggcggagtcctcagcgtcggagtctgagatctcccaggttggaggtcgccgctgaccgctcccgccccgtccccggccccggccctggcaagagacccccgccctcccgggtccaacccgcgccatggccggaccgacctcttcctcgcttccggccgcgaccgaacactttagcctgggacaccggcctcttccggtgacttccggccggaccgctgaggacgcggacccgccatggcgcggaagaaggtgcgtccgcggctgatcgcggagctggcccgccgcgtgcgcgccctgcgggagcaactgaacaggccgcgcgactcccagctctacgcggtggactacgagaccttgacgcggccgttctctggacgccggctgccggtccgggcctgggccgacgtgcgccgcgagagccgcctcttgcagctgctcggccgcctcccgctcttcggcctgggccgcctggtcacgcgcaagtcctggctgtggcagcacgacgagccgtgctactggcgcctcacgcgggtgcggcccgact

SEQ ID NO: 19051 - RNA, 223 nt, Homo sapiens
  source 1..223: mol_type = other RNA
tggcagttacttttgcaccagagcgattgtgcgtttgtttccgtataagtgcagtttatcaagccgaagctaagctacccaacgtttgctaagaagtactgtgtatttctggaaatttattcacaagtctgtgggaaatatgtttaattcttcttggaaatctcataaactctgaattcagtaccaccttccctgttttgtggcttatccttatccaccttct

SEQ ID NO: 19052 - RNA, 324 nt, Homo sapiens
  source 1..324: mol_type = other RNA
tggcagttacttttgcaccagagcgattgtgcgtttgtttccgtataagtgcagtttatcaagccgaagctaagctacccaacgtttgctaagaagtactgtgtatttctggaaatttattcacaagtctgtgggaaatatgtttaattcttcttggaaatctcataaactctgaattcagtaccaccttccctgttttgtggcttatccttatccaccttctttttcttcctatgagaaagtatttctttgctcattatgacttcagtagtgaagatgtaattttgcatcttcataagttaaaaataataaagtttgaacgca

SEQ ID NO: 19053 - RNA, 29 nt, Homo sapiens
  source 1..29: mol_type = other RNA
tggcagttacttttgcaccagcctaatat

SEQ ID NO: 19054 - RNA, 862 nt, Homo sapiens
  source 1..862: mol_type = other RNA
tggcagttacttttgcaccagcctaatattttctcaggccccaccccaggccaacagaatctatatctcaatggtgaagctcaagaatggacagctctgacaagtgcatcaggtgtttctgatgcccagtcgggtaggaaaatgacaaggttacatggatttggtctctttaaactataaacagttatgtttaatgagttgccaaggaactaaatacatagacatctgtaaccaggaataactttgtctcagataagccatctacgaataatcaggcaggcctgcaccttggcccaaaactccagacgttacctggtttccgacctagatgttagctgccaggctttgggtctgcctgctcacctgcccacctcccagattcctgatgcctgtcccctggtctggtatgattaccactgctcaagcctctctaaattcccggaagagattttctgaaaacaaaacatggtgtagaaaaatagtacaaaagaaacatgttctagaaatgaaaggtctatgttctaggagaagatttatgttccagaaacagaaattcctcctcctctgtatagatgtgcatcttgaaaaggtacttaaccagctactgttttgcactttcattatagtgctaagcactctgtgtttgctacatcatttaatcctttcttatattttgagatagggccattattattttatttacagatgagaacacaaaggctcagagagattgaataacttgtctaaggccagacagtgaacgaaaggcagaactgggattctaatttagtcttgactcttcacatctatgatggtgtttccccagtgtcctcatctgtaaaacaggaataatattggccag

SEQ ID NO: 19055 - RNA, 42 nt, Homo sapiens
  source 1..42: mol_type = other RNA
tggcagttacttttgcaccagctaactattcactggctgccc

SEQ ID NO: 19056 - RNA, 4597 nt, Homo sapiens
  source 1..4597: mol_type = other RNA
tggccaaaaagcaggcagagaaagggaggatgaagagattaatgcctacaaatatacagtttgaaagaagacctagtgttagatcagtagggtgtctatagtttacaataatctactgtgcatttcaaaatagctagaagagagtaatcataagaaagagccaaagggcagagcacaggatacagaaaagtgggatcaaatagagaagaatcccttagagttctgggtaggagcccaatctcaagtcttatttctaatgtttaaagctccccctactccccaaaatacctttagttggtgggattagttgtcctgtgaaaatctagacacaaaaattaggttggaaaagagaactcgtaactggaggccaatcatgctaggcattaaaaacgtattactgtattcctcctcctcctcatcagttgctaagtgacatttgggatttgaacccagtcctgatatctgaagctcacacactacacactgtattttctgctgtaaagcagacctcagaaagtatggttagattctgtgcaaccttgaaaatgctctggactcagtgggtccaactcagctatttgtacttcacaccacacagctagtctaggaaagaggctgcctctggcttgaccatgcaaatgtattttctttctttcctgccatgctggtcagcagttacaccaaagctagctagtatcagtatctgagtagatggtgatgacgacagagtctcagcatgcaacactagctactggcacactttgtttccagaggagttatggtgaatcttatactcaatgacaactgtattatgtaccgtactaaatagtaacggaaaacatgattccagtagagaaaaaccaagccatatagctgtctttcaatatgcttggtatgcagtgatatgcttgatagaaaatggtatgtctaatttttgaccataacttgaaacgtagagaatgagagagtgctcttaaaagcacatacatatacaacttggaagatgggacttacttggaaaagtacaaattattggaataatgaagtaatcttttaagctattttatataaggttaagatactatataaaataataatttttatcatatcatctgataaagcaagacaaaggaaaaaaaactgttttaagttagatcagcatttcccaaactgatactcaaaggaacattgtttcatgaaatgttaaaatatatgccttgaaaaaaattttatggatgaaagtttaaggaatagtatatcttaaaaatcttgggggtgggcaaaccaaaacttttttttttttttttccagtaagtaagtatgactatttctatttccaggagtgatctatgcaggagaaacagcttgggaaatgctgaaatttctgactgtaagaaatgcttggatatatgtatctgtttgtttggataatttactcatgtgatctcttggaaccaaggatccttggatccaaggaactctgatttctaggaatactttgtaaacaaatcaatatacaaataggtgaataatctgaattttccagcccagtgatttttgaaaggaggcatccaaaccaaaagagccccagatcagatttttacccaactaagtggtcagtgtttgtttatgacagtgaaccccctctgacagcttcatcacctctaacaaacaaacaaacaagggagacagagtggatgaacaacttattttcaaagctaacaaacattctatgacttaactgcttgaaaactaacttgttgcagaaaggtgaaatgctttattctcacagaaaactccacttctggagttgcccctcaatatgaagaaaccggaagtaaaagcctgtcattcttaaataacatttattattgttgcaaagaagtcttctccatgagaacagttctcacatttatttaaagatatagaggttatggatatagataagtatgcccgactatgatccttaattcagcaatctaatattcacaatgtgtttgttgccatttagctatttatcccaacatgcccttaaaaaaaacaccaaaaaaccacatgtgcctagacagggtggaaaaagaaacaccaaggccttgctaaaaaggagaagcctaaaaaagataaaattcccacggcagttctgttcaactgtagcctgtgagtgcaggaataatgttcccgtggggaagcattatgcccagtggtttcttggtgtcaacgtgggaaagcccttgaggttttctgtcgctgtcaggaggaagcacgaaaactgtttatggaatccagtcgacgttcaggcaccgcgcgatgaacgcaaacatgtctgagacttcctctatcactttggctgtgggcttccccgccccgtggcccgccttggtgtccacgtggataagcagggggttgctttgcttcctgctgcggcccacgatgtactgaagggtggcaatgaacttcagggagtgaagcgggaccacgcggtcatcatggtcagcagtgaggagcagcatggacgggtactggatgtcatctgcttctggtaacttcacattatgcaatggagagtatttgacaagccattcaaagtgttgtttgctgtccgagcacccataatcagtggtccaagcatggccgatggtatatttatgaaacttcagcatgtccattactccaacttgggcaataacacaaccaaagaggtcaggtctctgatttgcacaagcagccactaagaggcctccatttgaacctccattaatagtcagcctcttgggagatgtgtaaccttccttgatcagatactcagcagcacactgaaagtcatcaaagcagttttgtttgttggccaagataccacctttatgccacgtctctccatattcgccacctcctctgatgttggccactgccaggataccacccatgtgtctcacaaaaataagcctggaaacactgtagttgggtgtgatggatatgttgaagccgccatagccatataagaaagctggatgagagccatccaattttatgccttttttatgcacaatgaacattggaatcttcgtaccatccttgctagggtagaaaatctggactgtctggtaatcagaagcatcaattccttttacggtcacctctcggaaaactcttggctccagctcctctttggtaagatcacagtgataaatgatacctggagataaaaaggaagtaaactgatagaagatttcagtgtccttcttctgaccgctgtaccctacaatgctgccgacatcgagcgggaaggtcttaaggagagcaccagtagtcaggtcatggagctgcagaatgttcttgacgtcatggaggtagcataagaccaagaagttggacctgacacaagctatccattctaagacatctttctcatgctcaggaacaagtactttccacttagactcttcaggatccctgaagtcaatgttgatcacgcgatagttgggagactggcgattcgtcttgaatgtgaacaccgtcccctcattggtcacgtagtcatattccccttcaaagttgtcaatcagttttacccacttcaggattcccgcgatgccactggattcctgctgtaggtcacagtaccagagtcggtttactggatcacatccttcccttattgataacaagacatagcggccatcatcagataactcagctccacccatccatttaggttcatcaggaaactcagcacacaaaatatcttctgactgatcggttcccaagacatggtagtagagcttttggtggagattggtagatgtctctgtgccatcactttttccatcctgttgagggtatgagttgtagaacattcccttcccatcatgggtccaggccatacagctgaacttgactctttcaagcacatctggaagctctttggcaccatcaactttcatgaacttgattgtcacccagtctgagccactggcactcagaccataggcaaaatattcaccatcttcgctgaacgcataacctcggagtgccactgtgccatcgtcagacagtatgttggggtccaggaacactctggcctcaccctctaaggaatcctgtacatataatactcgctggttctgcaaacctgtattgtaaaaataaaaataccgttttcctttcttgaagtggcaactatacttgggataatcatatagttcagtcattctctctttgtataaacctctgatgggacactgctcaagaaatggcacagtaatcttattctgggcctccacaaaggccttagtctgttcactgtcggggtcttcaagccaggcgtaagggtcacaaattttatgaccatgataatcctgtacggcggtctcgtcgcggtacacgtcggggtactgaagggacagcatggccggggacaggcagggggcagcgtggaggggcgcgggctccgggagcggacctgagctagccgggctggccgcgaggcgcggctggggcgcaggcagctgcggggcggccggcggcagcgggcggccggctcacggccagagctagcacaaacggactggcggcgcggcggcgaggacgtgcagaaagc

SEQ ID NO: 19057 - RNA, 63 nt, Homo sapiens
  source 1..63: mol_type = other RNA
tggccaaaaagcaggcagagacgcttttaaagtctctgcctgctttttggccagctccatttt

SEQ ID NO: 19058 - RNA, 58 nt, Homo sapiens
  source 1..58: mol_type = other RNA
tggccaaaaagcaggcagagactttaaaagcgtctctgcctgctttttggccagctcc

SEQ ID NO: 19059 - RNA, 31 nt, Homo sapiens
  source 1..31: mol_type = other RNA
tggctcagttcagcaggaacaggagtcgagc

SEQ ID NO: 19060 - RNA, 567 nt, Homo sapiens
  source 1..567: mol_type = other RNA
tggctgttggagggggcaggcgtgtttccttgggaggaatgccgttacacaatcggtctgtcaagagtctgcgttcaggaatccaggcgaggtggctccagctgcggtctgctcctttgattcacacactccccacgggcagccccagccccttggctccctgctgcccttgggctgagtctcgatcccaaagctctctcccagaccctagtgaagaggaaagagtgaatgtatgagcaggcctgggtcccagactgtcttgctggctgctgtagtcacagtacctaacaaggggctagtatacagtacgttctcaataaatatgtgttaaatttatgaatgtttggggcattagaaacccaggtaccacctgggatgaggaagtgaggttccagaggagtggggagaaaaatatcagggtcatgatgggcattttggcctccttgaggggacccagaggaggaaggagctggtgctcctttccccatagagtggggagaagctccccctaggtctgccaaaggcatctcggcacacaggaagaaatgaggaatcaggggtcagaca

SEQ ID NO: 19061 - RNA, 77 nt, Homo sapiens
  source 1..77: mol_type = other RNA
tggcttttaactttgatggcaaagacatagattgtttagctacccctttgccatcaaagttaaaagccagagttaat

SEQ ID NO: 19062 - RNA, 77 nt, Homo sapiens
  source 1..77: mol_type = other RNA
tggcttttaactttgatggcaaaggggtagctaaacaatctatgtctttgccatcaaagttaaaagccatagttaat

SEQ ID NO: 19063 - RNA, 35 nt, Homo sapiens
  source 1..35: mol_type = other RNA
tgggaacttagtagaggtttaagttttaaatttgg

SEQ ID NO: 19064 - RNA, 6035 nt, Homo sapiens
  source 1..6035: mol_type = other RNA
tgggagagaggactgtgaggcttcaccaataaacctccctagagttcagctaccaatgaggttaataccgctactaaataacatgaacatctgcaaaagattcagagatataatgatgtttgcactcagctttgcatcgaataaataatgccatttctatgttaaatccttcccttgtcaccatagatcttccaatcaaacaaagagtataccatctaccaacataggtccttagtccttcgtaaactactatgttaattcaggttcttaagatttagtcaggcatttgcagaaacatcaatatggatatagtgctatgagaaaagagaggcaggttttataagaagagttaacaaggaaaatatagaaaataagatgatagtaatgctaaatttacatatttcccgattcttctggtgtagacaaactaagaaatccaatagttacttgggaggcacttgaaggtgtgagtatgtataatagagtgcctttattgtatgattggcttgcagaattcaaagatagttccttgtatgcatggtctcaagattaattattgtaacagttccataaggttattgatcattctttgatctcctagtgtataatacaccctaatcagaatgtaccattcagcaagttggattgattcttggtaatttttgagaaattcaccccatcgtttcagacgagaagtgtctggaatgacaaattcacagtagatcatttaatatgctatctccccttagagtgtgcattgtttaattattgattgtgtagatcactgatggttgcagctcatatttcaaaaagtatgtactggaagtctatgcacagcaaaatgtacacctaaaggggtatatgtttcagaatgggaaatggggctctatacttcaatttgtctcttttttggtaatatataagatgattcgtgaagtataatcattgaagatcaaggcgaagtttgtgataaacttcagaaaaacagaaatgtaaaccaataaaggactgatctaggtttgggcaaaatagtctcataagtatatttcatttgaggtattacagttgtaaattaaataataattttttgctgtgttaagaattttttttaatatatcaacagtttagttgaaaacattttacattctttgggaaactggcattactcagggtcttaagtactgtcaccatcaaacaatggtagcaaattaattggaaaactttttttaaaaggaaagacattacatactaacaaccactgcactttctgagtcttgttaaatacaacttgtatgttcagagttgaagtctgagactcaaaaccaaatgtattcaacattattaagaagagacaaatagaataatgagcaatacaaacaaagcaaagacagcaaaacatttttcaagactattgatgtattgtattgaatataatacagagaaaggcaaaggggctttattatgcttgtggccactgaagatgcaaacaccggccacacaggatctgagaagcatttccaggtctatgaataacaccacgaggagacaaaagcaaacacagcaaatgttctcaaataaagcaaggacattatagtccaaatttaatttttacctctaacaaaacttatgtattacatggttaagagaccaaggctacagttttcacatgtaaaaactgtagccattaagcaggttaaacttgttttagatcataccagaacagttgaaaattaacagcaatatctaatttcttgttccatagaatgaatgctatgagaaatatatcactggacgaggcttcctggagccaccccaagcctgtacatggcaagatggcagtgctgcaagcccactgcctgtacattcagtgtaagagcattcgtttttccattgagaacccctggctattaaaacaaactatcataattttatgttaaatcatagctgccaatcagaagaagtactctttctgattttcattgactgcattttgtatattaagctcacttttcagaacagcctcagcactgtctacattctctgacctttttgcctcacttcttttatataaccttttctgctgataaatgcgaacagctatggcagtgatgcaaagcaagataaaaatcacaacagctatcagacctccaattactgcagagtcacttttgattgcattagcaaggggctctctgtcatctattgttccagaatgatctgcaaacgagtgtgtcctttcccttgatgtggcatcagtgccaggctgggccatacagctggactcagtcacgtgtcctgccagtgcagtatcctggtccacatcactgtgttctaaaatcctgcccaataccagagatttgactgcactgaattctgtgcctgatgacaggtgaacttgtctccttctattatcgtcaatctctataaagaccactccttcttctctgttaatcattatgtggtgaagttgtccatcagccatgtttttaaaatcaaagttaacaacatcaggctcttgatatttatttaacttgtacctgatctgcaaacttccatttttggcaatgatcacagaaaggtattctttgtaaaaggagctcacaaaaagcagcaagcttggtgttcgtgttgttcggaaactaaatttgatcatttctctgctcagcttcatatcaccatgaaatgaagcagcgtgggagctggagtttttacttaaaagataattttcttgaaaattgtatatcacggatgagccagatccaaaatatgcagaaatctcatttgagcagaatggccctgtgtatgcagagaaagtgcagtcacaaaagaacccaatgggtctttctctgcatttccctccattgcggcataacttcccatagctgctgcaatgtcccctacaacctggctgcacttctggagtcacctgggctctttcttccaaatccagggtcatcccattcaactgcagagaccgaatgcagcccagaaagcctctctgtctggtggccgttccacccacgaagagctgactgttgagctgtaacaggacatgcccatcagcgggggcgggctgtgtctttggtgtcagctgatccacttgaagggaggcctccttcatgttcctttcaaccctcacatggtgccactggttgtcgttgaagtgggtgggtgactgcactgagatttcaaaaggcccattccccacatcaaatgaaaaagtcactactgtcggagagcgaagctctatccgtataaaatcagcaatccccaagttctctaaaaataccccagatgaagctgttgtcttaaaaaagaaagatacatccgcgctaagttctccgtggaaggtaggaaaatgaagatatgaagcctcggtatcaaaggaagctgaattccaaaatgatctgtctccctggcagagcagaggccccagtttataagctgcttctgaatgcagtcggcctgtgtctgtaatcacgatcttagttactggaagatgttctttataagcaagcaatccagtgtcattggtccattcattccggtcagcatcacaattgcagtaatactgagaatcaatgcagtttccctctaatccacaagtacatttttgaagatcaggcgaagaacctccccagtaggtttgcgtttcattggttcttcctacccaccaactcagaggggttccatcttgcttattgaccagccgtgacttcttgcagtaataagtaaactcctgttcacagtgctctgcacggttaatagtggcctgaagttgctccatgctggccacatactcgaaaaacccagcatatgggttctctggattagtatttctgactcttgttaagtcagagccgttgtgctgtatgatggtccatgcagtttcggtcatattgcaatatagaagaaatggttccaggggaccacttccatctgaatctatatagtaaaaccctgaagtatttcctctgtgcttataggcttcacatgactgctcatagatagagttatggcaagtagctcctctgtaaccagtgttggtacagttacaatgaaaggtgctccaggactgggaacactccccaccgtgttcacaatagttgggcaaacacctgtctgagatgccacatgagtctatctgaaggtcactgaagttcccaagggacccctgctgaactgaaatcagatctaccactttgccgctgatagaaatgagcctcatacatccctgaaatccaccaagtggacttttacatttggatccaaagcttttgtcaggacaacctccaaaataataggtgccacccgaataaatctgctcaggccccagcagaggagcagcagaagccatctggccgtccaccgccacactcaagtgattctttttagcagataaagagacagaatgccactgcccatcatttaattcgacacctgctgtgatgtcactgggtaattttcctggctggtagagattcgacttaagttttccatcactcagaaagaggaggataccccctgaaatcagctgaagttcactgaacagcagaagccctgccttattccaagttcgaaattgaaaagtggcagaaacctcctcctctccagagaagtctggcagtgctaaataactcctggagctcagaaaagtcacgggcatagattgtggttgtgaacaagaaaatgacacatttcccatagcaatgatctgtggtttttgctgcttggccaaatcaatgatatccactccattataatagagattttctaaacatccatgaaaatttctatgtgggaatgacactgattttccaggtgctggaatccctccaaagctgatctcataatcaagattcatgagattgaattctccccgtgcatggaaatgatgcctgtgttcgtccactgtgaagttgacttgtttgcccaaacgctggatgagcactgaatgccaatgctgatcatctagcaggctgcccagggtgagattgaccagggtggaagtggaaggcagtttagcttcacctgaattaataagtaaaaagagtcttgctcttcttaattgcagtgtgatgtgatctccatttggcccttccctgtggagtagaatcccatcactctgcatggttttgaatttcaaagaaataatgtcttttattgggctcagggatttttgatcaaatctgtagagaagggaactttttccatcaagatcaaccacttctgatctgtatgcacatccgaacacttcgattcgcattccaattctgcccttggggttccattccaaagggatgaagcgcagaaatctggctttgatagaaggctggagtctatagtacacaacactgtctgcatttgcatttcctgaaaaaccccagatgctgtcctcttggcgatattgtttccagttccagccactatcactgaacatcaggaggtagctggtcacccagttggagctaccatatcccccttgagtggccacagcggtgacctccattctctctccaaggtcaatctgcaaccactggtatttgttagacacaagtggagaccagccaccagctccatctcttctattcagccttgcaaatccaggaccatgactgctggagagctcggaagaactgctgaaggatgcctgaggcaaggcagacacaagaggatcatcacagtcataggaattcccagcttcgactctgttccaattttgagtagataacagaagtagcgtcttgaggacagctcccgtgacagatcccatgttcacatttattgggctcccccaaaagatcttgagaggctctcagagcgctccagtcctcttctcagtagctctgccagctctgtctgggtcttcagcccctctaggtctctgtctctccccctcccttcctcctcacctccctccgtcttttcttcttccctcctccctctcttctctctccctctctctctccccgtctctgtctctctcttttctctctctctctcacacacacctccctgactcctcactgaaaagc

SEQ ID NO: 19065 - RNA, 5941 nt, Homo sapiens
  source 1..5941: mol_type = other RNA
tgggagagaggactgtgaggcttcaccaataaacctccctagagttcagctaccaatgaggttaataccgctactaaataacatgaacatctgcaaaagattcagagatataatgatgtttgcactcagctttgcatcgaataaataatgccatttctatgttaaatccttcccttgtcaccatagatcttccaatcaaacaaagagtataccatctaccaacataggtccttagtccttcgtaaactactatgttaattcaggttcttaagatttagtcaggcatttgcagaaacatcaatatggatatagtgctatgagaaaagagaggcaggttttataagaagagttaacaaggaaaatatagaaaataagatgatagtaatgctaaatttacatatttcccgattcttctggtgtagacaaactaagaaatccaatagttacttgggaggcacttgaaggtgtgagtatgtataatagagtgcctttattgtatgattggcttgcagaattcaaagatagttccttgtatgcatggtctcaagattaattattgtaacagttccataaggttattgatcattctttgatctcctagtgtataatacaccctaatcagaatgtaccattcagcaagttggattgattcttggtaatttttgagaaattcaccccatcgtttcagacgagaagtgtctggaatgacaaattcacagtagatcatttaatatgctatctccccttagagtgtgcattgtttaattattgattgtgtagatcactgatggttgcagctcatatttcaaaaagtatgtactggaagtctatgcacagcaaaatgtacacctaaaggggtatatgtttcagaatgggaaatggggctctatacttcaatttgtctcttttttggtaatatataagatgattcgtgaagtataatcattgaagatcaaggcgaagtttgtgataaacttcagaaaaacagaaatgtaaaccaataaaggactgatctaggtttgggcaaaatagtctcataagtatatttcatttgaggtattacagttgtaaattaaataataattttttgctgtgttaagaattttttttaatatatcaacagtttagttgaaaacattttacattctttgggaaactggcattactcagggtcttaagtactgtcaccatcaaacaatggtagcaaattaattggaaaactttttttaaaaggaaagacattacatactaacaaccactgcactttctgagtcttgttaaatacaacttgtatgttcagagttgaagtctgagactcaaaaccaaatgtattcaacattattaagaagagacaaatagaataatgagcaatacaaacaaagcaaagacagcaaaacatttttcaagactattgatgtattgtattgaatataatacagagaaaggcaaaggggctttattatgcttgtggccactgaagatgcaaacaccggccacacaggatctgagaagcatttccaggtctatgaataacaccacgaggagacaaaagcaaacacagcaaatgttctcaaataaagcaaggacattatagtccaaatttaatttttacctctaacaaaacttatgtattacatggttaagagaccaaggctacagttttcacatgtaaaaactgtagccattaagcaggttaaacttgttttagatcataccagaacagttgaaaattaacagcaatatctaatttcttgttccatagaatgaatgctatgagaaatatatcactggacgaggcttcctggagccaccccaagcctgtacatggcaagatggcagtgctgcaagcccactgcctgtacattcagtgtaagagcattcgtttttccattgagaacccctggctattaaaacaaactatcataattttatgttaaatcatagctgccaatcagaagaagtactctttctgattttcattgactgcattttgtatattaagctcacttttcagaacagcctcagcactgtctacattctctgacctttttgcctcacttcttttatataaccttttctgctgataaatgcgaacagctatggcagtgatgcaaagcaagataaaaatcacaacagctatcagacctccaattactgcagagtcacttttgattgcattagcaaggggctctctgtcatctattgttccagaatgatctgcaaacgagtgtgtcctttcccttgatgtggcatcagtgccaggctgggccatacagctggactcagtcacgtgtcctgtaacagtgacagggtctgggtggctggggtgcagagctgccttcagaggggccacgtggctgagctgcactgcagagaggcagcctgtgaagccctgcgcacctgccagtgcagtatcctggtccacatcactgtgttctaaaatcctgcccaataccagagatttgactgcactgaattctgtgcctgatgacaggtgaacttgtctccttctattatcgtcaatctctataaagaccactccttcttctctgttaatcattatgtggtgaagttgtccatcagccatgtttttaaaatcaaagttaacaacatcaggctcttgatatttatttaacttgtacctgatctgcaaacttccatttttggcaatgatcacagaaaggtattctttgtaaaaggagctcacaaaaagcagcaagcttggtgttcgtgttgttcggaaactaaatttgatcatttctctgctcagcttcatatcaccatgaaatgaagcagcgtgggagctggagtttttacttaaaagataattttcttgaaaattgtatatcacggatgagccagatccaaaatatgcagaaatctcatttgagcagaatggccctgtgtatgcagagaaagtgcagtcacaaaagaacccaatgggtctttctctgcatttccctccattgcggcataacttcccatagctgctgcaatgtcccctacaacctggctgcacttctggagtcacctgggctctttcttccaaatccagggtcatcccattcaactgcagagaccgaatgcagcccagaaagcctctctgtctggtggccgttccacccacgaagagctgactgttgagctgtaacaggacatgcccatcagcgggggcgggctgtgtctttggtgtcagctgatccacttgaagggaggcctccttcatgttcctttcaaccctcacatggtgccactggttgtcgttgaagtgggtgggtgactgcactgagatttcaaaaggcccattccccacatcaaatgaaaaagtcactactgtcggagagcgaagctctatccgtataaaatcagcaatccccaagttctctaaaaataccccagatgaagctgttgtcttaaaaaagaaagatacatccgcgctaagttctccgtggaaggtaggaaaatgaagatatgaagcctcggtatcaaaggaagctgaattccaaaatgatctgtctccctggcagagcagaggccccagtttataagctgcttctgaatgcagtcggcctgtgtctgtaatcacgatcttagttactggaagatgttctttataagcaagcaatccagtgtcattggtccattcattccggtcagcatcacaattgcagtaatactgagaatcaatgcagtttccctctaatccacaagtacatttttgaagatcaggcgaagaacctccccagtaggtttgcgtttcattggttcttcctacccaccaactcagaggggttccatcttgcttattgaccagccgtgacttcttgcagtaataagtaaactcctgttcacagtgctctgcacggttaatagtggcctgaagttgctccatgctggccacatactcgaaaaacccagcatatgggttctctggattagtatttctgactcttgttaagtcagagccgttgtgctgtatgatggtccatgcagtttcggtcatattgcaatatagaagaaatggttccaggggaccacttccatctgaatctatatagtaaaaccctgaagtatttcctctgtgcttataggcttcacatgactgctcatagatagagttatggcaagtagctcctctgtaaccagtgttggtacagttacaatgaaaggtgctccaggactgggaacactccccaccgtgttcacaatagttgggcaaacacctgtctgagatgccacatgagtctatctgaaggtcactgaagttcccaagggacccctgctgaactgaaatcagatctaccactttgccgctgatagaaatgagcctcatacatccctgaaatccaccaagtggacttttacatttggatccaaagcttttgtcaggacaacctccaaaataataggtgccacccgaataaatctgctcaggccccagcagaggagcagcagaagccatctggccgtccaccgccacactcaagtgattctttttagcagataaagagacagaatgccactgcccatcatttaattcgacacctgctgtgatgtcactgggtaattttcctggctggtagagattcgacttaagttttccatcactcagaaagaggaggataccccctgaaatcagctgaagttcactgaacagcagaagccctgccttattccaagttcgaaattgaaaagtggcagaaacctcctcctctccagagaagtctggcagtgctaaataactcctggagctcagaaaagtcacgggcatagattgtggttgtgaacaagaaaatgacacatttcccatagcaatgatctgtggtttttgctgcttggccaaatcaatgatatccactccattataatagagattttctaaacatccatgaaaatttctatgtgggaatgacactgattttccaggtgctggaatccctccaaagctcataatcaagattcatgagattgaattctccccgtgcatggaaatgatgcctgtgttcgtccactgtgaagttgacttgtttgcccaaacgctggatgagcactgaatgccaatgctgatcatctagcaggctgcccagggtgagattgaccagggtggaagtggaaggcagtttagcttcacctgaattaataagtaaaaagagtcttgctcttcttaattgcagtgtgatgtgatctccatttggcccttccctgtggagtagaatcccatcactctgcatggttttgaatttcaaagaaataatgtcttttattgggctcagggatttttgatcaaatctgtagagaagggaactttttccatcaagatcaaccacttctgatctgtatgcacatccgaacacttcgattcgcattccaattctgcccttggggttccattccaaagggatgaagcgcagaaatctggctttgatagaaggctggagtctatagtacacaacactgtctgcatttgcatttcctgaaaaacccatctcttctattcagccttgcaaatccaggaccatgactgctggagagctcggaagaactgctgaaggatgcctgaggcaaggcagacacaagaggatcatcacagtcataggaattcccagcttcgactctgttccaattttgagtagataacagaagtagcgtcttgaggacagctcccgtgacagatcccatgttcacatttattgggctcccccaaaagatcttgagaggctctcagagcgctccagtcctcttctcagtagctctgccagctctgtctgggtcttcagcccctctaggtctctgtctctccccctcccttcctcctcacctccctccgtcttttcttcttccctcctccctctcttctctctccctctctctctccccgtctctgtctctctcttttctctctctctctcacacacacctccctgactcctcactgaaaagc

SEQ ID NO: 19066 - RNA, 6133 nt, Homo sapiens
  source 1..6133: mol_type = other RNA
tgggagagaggactgtgaggcttcaccaataaacctccctagagttcagctaccaatgaggttaataccgctactaaataacatgaacatctgcaaaagattcagagatataatgatgtttgcactcagctttgcatcgaataaataatgccatttctatgttaaatccttcccttgtcaccatagatcttccaatcaaacaaagagtataccatctaccaacataggtccttagtccttcgtaaactactatgttaattcaggttcttaagatttagtcaggcatttgcagaaacatcaatatggatatagtgctatgagaaaagagaggcaggttttataagaagagttaacaaggaaaatatagaaaataagatgatagtaatgctaaatttacatatttcccgattcttctggtgtagacaaactaagaaatccaatagttacttgggaggcacttgaaggtgtgagtatgtataatagagtgcctttattgtatgattggcttgcagaattcaaagatagttccttgtatgcatggtctcaagattaattattgtaacagttccataaggttattgatcattctttgatctcctagtgtataatacaccctaatcagaatgtaccattcagcaagttggattgattcttggtaatttttgagaaattcaccccatcgtttcagacgagaagtgtctggaatgacaaattcacagtagatcatttaatatgctatctccccttagagtgtgcattgtttaattattgattgtgtagatcactgatggttgcagctcatatttcaaaaagtatgtactggaagtctatgcacagcaaaatgtacacctaaaggggtatatgtttcagaatgggaaatggggctctatacttcaatttgtctcttttttggtaatatataagatgattcgtgaagtataatcattgaagatcaaggcgaagtttgtgataaacttcagaaaaacagaaatgtaaaccaataaaggactgatctaggtttgggcaaaatagtctcataagtatatttcatttgaggtattacagttgtaaattaaataataattttttgctgtgttaagaattttttttaatatatcaacagtttagttgaaaacattttacattctttgggaaactggcattactcagggtcttaagtactgtcaccatcaaacaatggtagcaaattaattggaaaactttttttaaaaggaaagacattacatactaacaaccactgcactttctgagtcttgttaaatacaacttgtatgttcagagttgaagtctgagactcaaaaccaaatgtattcaacattattaagaagagacaaatagaataatgagcaatacaaacaaagcaaagacagcaaaacatttttcaagactattgatgtattgtattgaatataatacagagaaaggcaaaggggctttattatgcttgtggccactgaagatgcaaacaccggccacacaggatctgagaagcatttccaggtctatgaataacaccacgaggagacaaaagcaaacacagcaaatgttctcaaataaagcaaggacattatagtccaaatttaatttttacctctaacaaaacttatgtattacatggttaagagaccaaggctacagttttcacatgtaaaaactgtagccattaagcaggttaaacttgttttagatcataccagaacagttgaaaattaacagcaatatctaatttcttgttccatagaatgaatgctatgagaaatatatcactggacgaggcttcctggagccaccccaagcctgtacatggcaagatggcagtgctgcaagcccactgcctgtacattcagtgtaagagcattcgtttttccattgagaacccctggctattaaaacaaactatcataattttatgttaaatcatagctgccaatcagaagaagtactctttctgattttcattgactgcattttgtatattaagctcacttttcagaacagcctcagcactgtctacattctctgacctttttgcctcacttcttttatataaccttttctgctgataaatgcgaacagctatggcagtgatgcaaagcaagataaaaatcacaacagctatcagacctccaattactgcagagtcacttttgattgcattagcaaggggctctctgtcatctattgttccagaatgatctgcaaacgagtgtgtcctttcccttgatgtggcatcagtgccaggctgggccatacagctggactcagtcacgtgtcctgtaacagtgacagggtctgggtggctggggtgcagagctgccttcagaggggccacgtggctgagctgcactgcagagaggcagcctgtgaagccctgcgcacctgccagtgcagtatcctggtccacatcactgtgttctaaaatcctgcccaataccagagatttgactgcactgaattctgtgcctgatgacaggtgaacttgtctccttctattatcgtcaatctctataaagaccactccttcttctctgttaatcattatgtggtgaagttgtccatcagccatgtttttaaaatcaaagttaacaacatcaggctcttgatatttatttaacttgtacctgatctgcaaacttccatttttggcaatgatcacagaaaggtattctttgtaaaaggagctcacaaaaagcagcaagcttggtgttcgtgttgttcggaaactaaatttgatcatttctctgctcagcttcatatcaccatgaaatgaagcagcgtgggagctggagtttttacttaaaagataattttcttgaaaattgtatatcacggatgagccagatccaaaatatgcagaaatctcatttgagcagaatggccctgtgtatgcagagaaagtgcagtcacaaaagaacccaatgggtctttctctgcatttccctccattgcggcataacttcccatagctgctgcaatgtcccctacaacctggctgcacttctggagtcacctgggctctttcttccaaatccagggtcatcccattcaactgcagagaccgaatgcagcccagaaagcctctctgtctggtggccgttccacccacgaagagctgactgttgagctgtaacaggacatgcccatcagcgggggcgggctgtgtctttggtgtcagctgatccacttgaagggaggcctccttcatgttcctttcaaccctcacatggtgccactggttgtcgttgaagtgggtgggtgactgcactgagatttcaaaaggcccattccccacatcaaatgaaaaagtcactactgtcggagagcgaagctctatccgtataaaatcagcaatccccaagttctctaaaaataccccagatgaagctgttgtcttaaaaaagaaagatacatccgcgctaagttctccgtggaaggtaggaaaatgaagatatgaagcctcggtatcaaaggaagctgaattccaaaatgatctgtctccctggcagagcagaggccccagtttataagctgcttctgaatgcagtcggcctgtgtctgtaatcacgatcttagttactggaagatgttctttataagcaagcaatccagtgtcattggtccattcattccggtcagcatcacaattgcagtaatactgagaatcaatgcagtttccctctaatccacaagtacatttttgaagatcaggcgaagaacctccccagtaggtttgcgtttcattggttcttcctacccaccaactcagaggggttccatcttgcttattgaccagccgtgacttcttgcagtaataagtaaactcctgttcacagtgctctgcacggttaatagtggcctgaagttgctccatgctggccacatactcgaaaaacccagcatatgggttctctggattagtatttctgactcttgttaagtcagagccgttgtgctgtatgatggtccatgcagtttcggtcatattgcaatatagaagaaatggttccaggggaccacttccatctgaatctatatagtaaaaccctgaagtatttcctctgtgcttataggcttcacatgactgctcatagatagagttatggcaagtagctcctctgtaaccagtgttggtacagttacaatgaaaggtgctccaggactgggaacactccccaccgtgttcacaatagttgggcaaacacctgtctgagatgccacatgagtctatctgaaggtcactgaagttcccaagggacccctgctgaactgaaatcagatctaccactttgccgctgatagaaatgagcctcatacatccctgaaatccaccaagtggacttttacatttggatccaaagcttttgtcaggacaacctccaaaataataggtgccacccgaataaatctgctcaggccccagcagaggagcagcagaagccatctggccgtccaccgccacactcaagtgattctttttagcagataaagagacagaatgccactgcccatcatttaattcgacacctgctgtgatgtcactgggtaattttcctggctggtagagattcgacttaagttttccatcactcagaaagaggaggataccccctgaaatcagctgaagttcactgaacagcagaagccctgccttattccaagttcgaaattgaaaagtggcagaaacctcctcctctccagagaagtctggcagtgctaaataactcctggagctcagaaaagtcacgggcatagattgtggttgtgaacaagaaaatgacacatttcccatagcaatgatctgtggtttttgctgcttggccaaatcaatgatatccactccattataatagagattttctaaacatccatgaaaatttctatgtgggaatgacactgattttccaggtgctggaatccctccaaagctcataatcaagattcatgagattgaattctccccgtgcatggaaatgatgcctgtgttcgtccactgtgaagttgacttgtttgcccaaacgctggatgagcactgaatgccaatgctgatcatctagcaggctgcccagggtgagattgaccagggtggaagtggaaggcagtttagcttcacctgaattaataagtaaaaagagtcttgctcttcttaattgcagtgtgatgtgatctccatttggcccttccctgtggagtagaatcccatcactctgcatggttttgaatttcaaagaaataatgtcttttattgggctcagggatttttgatcaaatctgtagagaagggaactttttccatcaagatcaaccacttctgatctgtatgcacatccgaacacttcgattcgcattccaattctgcccttggggttccattccaaagggatgaagcgcagaaatctggctttgatagaaggctggagtctatagtacacaacactgtctgcatttgcatttcctgaaaaaccccagatgctgtcctcttggcgatattgtttccagttccagccactatcactgaacatcaggaggtagctggtcacccagttggagctaccatatcccccttgagtggccacagcggtgacctccattctctctccaaggtcaatctgcaaccactggtatttgttagacacaagtggagaccagccaccagctccatctcttctattcagccttgcaaatccaggaccatgactgctggagagctcggaagaactgctgaaggatgcctgaggcaaggcagacacaagaggatcatcacagtcataggaattcccagcttcgactctgttccaattttgagtagataacagaagtagcgtcttgaggacagctcccgtgacagatcccatgttcacatttattgggctcccccaaaagatcttgagaggctctcagagcgctccagtcctcttctcagtagctctgccagctctgtctgggtcttcagcccctctaggtctctgtctctccccctcccttcctcctcacctccctccgtcttttcttcttccctcctccctctcttctctctccctctctctctccccgtctctgtctctctcttttctctctctctctcacacacacctccctgactcctcactgaaaa

SEQ ID NO: 19067 - RNA, 5946 nt, Homo sapiens
  source 1..5946: mol_type = other RNA
tgggagagaggactgtgaggcttcaccaataaacctccctagagttcagctaccaatgaggttaataccgctactaaataacatgaacatctgcaaaagattcagagatataatgatgtttgcactcagctttgcatcgaataaataatgccatttctatgttaaatccttcccttgtcaccatagatcttccaatcaaacaaagagtataccatctaccaacataggtccttagtccttcgtaaactactatgttaattcaggttcttaagatttagtcaggcatttgcagaaacatcaatatggatatagtgctatgagaaaagagaggcaggttttataagaagagttaacaaggaaaatatagaaaataagatgatagtaatgctaaatttacatatttcccgattcttctggtgtagacaaactaagaaatccaatagttacttgggaggcacttgaaggtgtgagtatgtataatagagtgcctttattgtatgattggcttgcagaattcaaagatagttccttgtatgcatggtctcaagattaattattgtaacagttccataaggttattgatcattctttgatctcctagtgtataatacaccctaatcagaatgtaccattcagcaagttggattgattcttggtaatttttgagaaattcaccccatcgtttcagacgagaagtgtctggaatgacaaattcacagtagatcatttaatatgctatctccccttagagtgtgcattgtttaattattgattgtgtagatcactgatggttgcagctcatatttcaaaaagtatgtactggaagtctatgcacagcaaaatgtacacctaaaggggtatatgtttcagaatgggaaatggggctctatacttcaatttgtctcttttttggtaatatataagatgattcgtgaagtataatcattgaagatcaaggcgaagtttgtgataaacttcagaaaaacagaaatgtaaaccaataaaggactgatctaggtttgggcaaaatagtctcataagtatatttcatttgaggtattacagttgtaaattaaataataattttttgctgtgttaagaattttttttaatatatcaacagtttagttgaaaacattttacattctttgggaaactggcattactcagggtcttaagtactgtcaccatcaaacaatggtagcaaattaattggaaaactttttttaaaaggaaagacattacatactaacaaccactgcactttctgagtcttgttaaatacaacttgtatgttcagagttgaagtctgagactcaaaaccaaatgtattcaacattattaagaagagacaaatagaataatgagcaatacaaacaaagcaaagacagcaaaacatttttcaagactattgatgtattgtattgaatataatacagagaaaggcaaaggggctttattatgcttgtggccactgaagatgcaaacaccggccacacaggatctgagaagcatttccaggtctatgaataacaccacgaggagacaaaagcaaacacagcaaatgttctcaaataaagcaaggacattatagtccaaatttaatttttacctctaacaaaacttatgtattacatggttaagagaccaaggctacagttttcacatgtaaaaactgtagccattaagcaggttaaacttgttttagatcataccagaacagttgaaaattaacagcaatatctaatttcttgttccatagaatgaatgctatgagaaatatatcactggacgaggcttcctggagccaccccaagcctgtacatggcaagatggcagtgctgcaagcccactgcctgtacattcagtgtaagagcattcgtttttccattgagaacccctggctattaaaacaaactatcataattttatgttaaatcatagctgccaatcagaagaagtactctttctgattttcattgactgcattttgtatattaagctcacttttcagaacagcctcagcactgtctacattctctgacctttttgcctcacttcttttatataaccttttctgctgataaatgcgaacagctatggcagtgatgcaaagcaagataaaaatcacaacagctatcagacctccaattactgcagagtcacttttgattgcattagcaaggggctctctgtcatctattgttccagaatgatctgcaaacgagtgtgtcctttcccttgatgtggcatcagtgccaggctgggccatacagctggactcagtcacgtgtcctgtaacagtgacagggtctgggtggctggggtgcagagctgccttcagaggggccacgtggctgagctgcactgcagagaggcagcctgtgaagccctgcgcacctgccagtgcagtatcctggtccacatcactgtgttctaaaatcctgcccaataccagagatttgactgcactgaattctgtgcctgatgacaggtgaacttgtctccttctattatcgtcaatctctataaagaccactccttcttctctgttaatcattatgtggtgaagttgtccatcagccatgtttttaaaatcaaagttaacaacatcaggctcttgatatttatttaacttgtacctgatctgcaaacttccatttttggcaatgatcacagaaaggtattctttgtaaaaggagctcacaaaaagcagcaagcttggtgttcgtgttgttcggaaactaaatttgatcatttctctgctcagcttcatatcaccatgaaatgaagcagcgtgggagctggagtttttacttaaaagataattttcttgaaaattgtatatcacggatgagccagatccaaaatatgcagaaatctcatttgagcagaatggccctgtgtatgcagagaaagtgcagtcacaaaagaacccaatgggtctttctctgcatttccctccattgcggcataacttcccatagctgctgcaatgtcccctacaacctggctgcacttctggagtcacctgggctctttcttccaaatccagggtcatcccattcaactgcagagaccgaatgcagcccagaaagcctctctgtctggtggccgttccacccacgaagagctgactgttgagctgtaacaggacatgcccatcagcgggggcgggctgtgtctttggtgtcagctgatccacttgaagggaggcctccttcatgttcctttcaaccctcacatggtgccactggttgtcgttgaagtgggtgggtgactgcactgagatttcaaaaggcccattccccacatcaaatgaaaaagtcactactgtcggagagcgaagctctatccgtataaaatcagcaatccccaagttctctaaaaataccccagatgaagctgttgtcttaaaaaagaaagatacatccgcgctaagttctccgtggaaggtaggaaaatgaagatatgaagcctcggtatcaaaggaagctgaattccaaaatgatctgtctccctggcagagcagaggccccagtttataagctgcttctgaatgcagtcggcctgtgtctgtaatcacgatcttagttactggaagatgttctttataagcaagcaatccagtgtcattggtccattcattccggtcagcatcacaattgcagtaatactgagaatcaatgcagtttccctctaatccacaagtacatttttgaagatcaggcgaagaacctccccagtaggtttgcgtttcattggttcttcctacccaccaactcagaggggttccatcttgcttattgaccagccgtgacttcttgcagtaataagtaaactcctgttcacagtgctctgcacggttaatagtggcctgaagttgctccatgctggccacatactcgaaaaacccagcatatgggttctctggattagtatttctgactcttgttaagtcagagccgttgtgctgtatgatggtccatgcagtttcggtcatattgcaatatagaagaaatggttccaggggaccacttccatctgaatctatatagtaaaaccctgaagtatttcctctgtgcttataggcttcacatgactgctcatagatagagttatggcaagtagctcctctgtaaccagtgttggtacagttacaatgaaaggtgctccaggactgggaacactccccaccgtgttcacaatagttgggcaaacacctgtctgagatgccacatgagtctatctgaaggtcactgaagttcccaagggacccctgctgaactgaaatcagatctaccactttgccgctgatagaaatgagcctcatacatccctgaaatccaccaagtggacttttacatttggatccaaagcttttgtcaggacaacctccaaaataataggtgccacccgaataaatctgctcaggccccagcagaggagcagcagaagccatctggccgtccaccgccacactcaagtgattctttttagcagataaagagacagaatgccactgcccatcatttaattcgacacctgctgtgatgtcactgggtaattttcctggctggtagagattcgacttaagttttccatcactcagaaagaggaggataccccctgaaatcagctgaagttcactgaacagcagaagccctgccttattccaagttcgaaattgaaaagtggcagaaacctcctcctctccagagaagtctggcagtgctaaataactcctggagctcagaaaagtcacgggcatagattgtggttgtgaacaagaaaatgacacatttcccatagcaatgatctgtggtttttgctgcttggccaaatcaatgatatccactccattataatagagattttctaaacatccatgaaaatttctatgtgggaatgacactgattttccaggtgctggaatccctccaaagctgatctcataatcaagattcatgagattgaattctccccgtgcatggaaatgatgcctgtgttcgtccactgtgaagttgacttgtttgcccaaacgctggatgagcactgaatgccaatgctgatcatctagcaggctgcccagggtgagattgaccagggtggaagtggaaggcagtttagcttcacctgaattaataagtaaaaagagtcttgctcttcttaattgcagtgtgatgtgatctccatttggcccttccctgtggagtagaatcccatcactctgcatggttttgaatttcaaagaaataatgtcttttattgggctcagggatttttgatcaaatctgtagagaagggaactttttccatcaagatcaaccacttctgatctgtatgcacatccgaacacttcgattcgcattccaattctgcccttggggttccattccaaagggatgaagcgcagaaatctggctttgatagaaggctggagtctatagtacacaacactgtctgcatttgcatttcctgaaaaacccatctcttctattcagccttgcaaatccaggaccatgactgctggagagctcggaagaactgctgaaggatgcctgaggcaaggcagacacaagaggatcatcacagtcataggaattcccagcttcgactctgttccaattttgagtagataacagaagtagcgtcttgaggacagctcccgtgacagatcccatgttcacatttattgggctcccccaaaagatcttgagaggctctcagagcgctccagtcctcttctcagtagctctgccagctctgtctgggtcttcagcccctctaggtctctgtctctccccctcccttcctcctcacctccctccgtcttttcttcttccctcctccctctcttctctctccctctctctctccccgtctctgtctctctcttttctctctctctctcacacacacctccctgactcctcactgaaaagc

SEQ ID NO: 19068 - RNA, 6137 nt, Homo sapiens
  source 1..6137: mol_type = other RNA
tgggagagaggactgtgaggcttcaccaataaacctccctagagttcagctaccaatgaggttaataccgctactaaataacatgaacatctgcaaaagattcagagatataatgatgtttgcactcagctttgcatcgaataaataatgccatttctatgttaaatccttcccttgtcaccatagatcttccaatcaaacaaagagtataccatctaccaacataggtccttagtccttcgtaaactactatgttaattcaggttcttaagatttagtcaggcatttgcagaaacatcaatatggatatagtgctatgagaaaagagaggcaggttttataagaagagttaacaaggaaaatatagaaaataagatgatagtaatgctaaatttacatatttcccgattcttctggtgtagacaaactaagaaatccaatagttacttgggaggcacttgaaggtgtgagtatgtataatagagtgcctttattgtatgattggcttgcagaattcaaagatagttccttgtatgcatggtctcaagattaattattgtaacagttccataaggttattgatcattctttgatctcctagtgtataatacaccctaatcagaatgtaccattcagcaagttggattgattcttggtaatttttgagaaattcaccccatcgtttcagacgagaagtgtctggaatgacaaattcacagtagatcatttaatatgctatctccccttagagtgtgcattgtttaattattgattgtgtagatcactgatggttgcagctcatatttcaaaaagtatgtactggaagtctatgcacagcaaaatgtacacctaaaggggtatatgtttcagaatgggaaatggggctctatacttcaatttgtctcttttttggtaatatataagatgattcgtgaagtataatcattgaagatcaaggcgaagtttgtgataaacttcagaaaaacagaaatgtaaaccaataaaggactgatctaggtttgggcaaaatagtctcataagtatatttcatttgaggtattacagttgtaaattaaataataattttttgctgtgttaagaattttttttaatatatcaacagtttagttgaaaacattttacattctttgggaaactggcattactcagggtcttaagtactgtcaccatcaaacaatggtagcaaattaattggaaaactttttttaaaaggaaagacattacatactaacaaccactgcactttctgagtcttgttaaatacaacttgtatgttcagagttgaagtctgagactcaaaaccaaatgtattcaacattattaagaagagacaaatagaataatgagcaatacaaacaaagcaaagacagcaaaacatttttcaagactattgatgtattgtattgaatataatacagagaaaggcaaaggggctttattatgcttgtggccactgaagatgcaaacaccggccacacaggatctgagaagcatttccaggtctatgaataacaccacgaggagacaaaagcaaacacagcaaatgttctcaaataaagcaaggacattatagtccaaatttaatttttacctctaacaaaacttatgtattacatggttaagagaccaaggctacagttttcacatgtaaaaactgtagccattaagcaggttaaacttgttttagatcataccagaacagttgaaaattaacagcaatatctaatttcttgttccatagaatgaatgctatgagaaatatatcactggacgaggcttcctggagccaccccaagcctgtacatggcaagatggcagtgctgcaagcccactgcctgtacattcagtgtaagagcattcgtttttccattgagaacccctggctattaaaacaaactatcataattttatgttaaatcatagctgccaatcagaagaagtactctttctgattttcattgactgcattttgtatattaagctcacttttcagaacagcctcagcactgtctacattctctgacctttttgcctcacttcttttatataaccttttctgctgataaatgcgaacagctatggcagtgatgcaaagcaagataaaaatcacaacagctatcagacctccaattactgcagagtcacttttgattgcattagcaaggggctctctgtcatctattgttccagaatgatctgcaaacgagtgtgtcctttcccttgatgtggcatcagtgccaggctgggccatacagctggactcagtcacgtgtcctgtaacagtgacagggtctgggtggctggggtgcagagctgccttcagaggggccacgtggctgagctgcactgcagagaggcagcctgtgaagccctgcgcacctgccagtgcagtatcctggtccacatcactgtgttctaaaatcctgcccaataccagagatttgactgcactgaattctgtgcctgatgacaggtgaacttgtctccttctattatcgtcaatctctataaagaccactccttcttctctgttaatcattatgtggtgaagttgtccatcagccatgtttttaaaatcaaagttaacaacatcaggctcttgatatttatttaacttgtacctgatctgcaaacttccatttttggcaatgatcacagaaaggtattctttgtaaaaggagctcacaaaaagcagcaagcttggtgttcgtgttgttcggaaactaaatttgatcatttctctgctcagcttcatatcaccatgaaatgaagcagcgtgggagctggagtttttacttaaaagataattttcttgaaaattgtatatcacggatgagccagatccaaaatatgcagaaatctcatttgagcagaatggccctgtgtatgcagagaaagtgcagtcacaaaagaacccaatgggtctttctctgcatttccctccattgcggcataacttcccatagctgctgcaatgtcccctacaacctggctgcacttctggagtcacctgggctctttcttccaaatccagggtcatcccattcaactgcagagaccgaatgcagcccagaaagcctctctgtctggtggccgttccacccacgaagagctgactgttgagctgtaacaggacatgcccatcagcgggggcgggctgtgtctttggtgtcagctgatccacttgaagggaggcctccttcatgttcctttcaaccctcacatggtgccactggttgtcgttgaagtgggtgggtgactgcactgagatttcaaaaggcccattccccacatcaaatgaaaaagtcactactgtcggagagcgaagctctatccgtataaaatcagcaatccccaagttctctaaaaataccccagatgaagctgttgtcttaaaaaagaaagatacatccgcgctaagttctccgtggaaggtaggaaaatgaagatatgaagcctcggtatcaaaggaagctgaattccaaaatgatctgtctccctggcagagcagaggccccagtttataagctgcttctgaatgcagtcggcctgtgtctgtaatcacgatcttagttactggaagatgttctttataagcaagcaatccagtgtcattggtccattcattccggtcagcatcacaattgcagtaatactgagaatcaatgcagtttccctctaatccacaagtacatttttgaagatcaggcgaagaacctccccagtaggtttgcgtttcattggttcttcctacccaccaactcagaggggttccatcttgcttattgaccagccgtgacttcttgcagtaataagtaaactcctgttcacagtgctctgcacggttaatagtggcctgaagttgctccatgctggccacatactcgaaaaacccagcatatgggttctctggattagtatttctgactcttgttaagtcagagccgttgtgctgtatgatggtccatgcagtttcggtcatattgcaatatagaagaaatggttccaggggaccacttccatctgaatctatatagtaaaaccctgaagtatttcctctgtgcttataggcttcacatgactgctcatagatagagttatggcaagtagctcctctgtaaccagtgttggtacagttacaatgaaaggtgctccaggactgggaacactccccaccgtgttcacaatagttgggcaaacacctgtctgagatgccacatgagtctatctgaaggtcactgaagttcccaagggacccctgctgaactgaaatcagatctaccactttgccgctgatagaaatgagcctcatacatccctgaaatccaccaagtggacttttacatttggatccaaagcttttgtcaggacaacctccaaaataataggtgccacccgaataaatctgctcaggccccagcagaggagcagcagaagccatctggccgtccaccgccacactcaagtgattctttttagcagataaagagacagaatgccactgcccatcatttaattcgacacctgctgtgatgtcactgggtaattttcctggctggtagagattcgacttaagttttccatcactcagaaagaggaggataccccctgaaatcagctgaagttcactgaacagcagaagccctgccttattccaagttcgaaattgaaaagtggcagaaacctcctcctctccagagaagtctggcagtgctaaataactcctggagctcagaaaagtcacgggcatagattgtggttgtgaacaagaaaatgacacatttcccatagcaatgatctgtggtttttgctgcttggccaaatcaatgatatccactccattataatagagattttctaaacatccatgaaaatttctatgtgggaatgacactgattttccaggtgctggaatccctccaaagctgatctcataatcaagattcatgagattgaattctccccgtgcatggaaatgatgcctgtgttcgtccactgtgaagttgacttgtttgcccaaacgctggatgagcactgaatgccaatgctgatcatctagcaggctgcccagggtgagattgaccagggtggaagtggaaggcagtttagcttcacctgaattaataagtaaaaagagtcttgctcttcttaattgcagtgtgatgtgatctccatttggcccttccctgtggagtagaatcccatcactctgcatggttttgaatttcaaagaaataatgtcttttattgggctcagggatttttgatcaaatctgtagagaagggaactttttccatcaagatcaaccacttctgatctgtatgcacatccgaacacttcgattcgcattccaattctgcccttggggttccattccaaagggatgaagcgcagaaatctggctttgatagaaggctggagtctatagtacacaacactgtctgcatttgcatttcctgaaaaaccccagatgctgtcctcttggcgatattgtttccagttccagccactatcactgaacatcaggaggtagctggtcacccagttggagctaccatatcccccttgagtggccacagcggtgacctccattctctctccaaggtcaatctgcaaccactggtatttgttagacacaagtggagaccagccaccagcatctcttctattcagccttgcaaatccaggaccatgactgctggagagctcggaagaactgctgaaggatgcctgaggcaaggcagacacaagaggatcatcacagtcataggaattcccagcttcgactctgttccaattttgagtagataacagaagtagcgtcttgaggacagctcccgtgacagatcccatgttcacatttattgggctcccccaaaagatcttgagaggctctcagagcgctccagtcctcttctcagtagctctgccagctctgtctgggtcttcagcccctctaggtctctgtctctccccctcccttcctcctcacctccctccgtcttttcttcttccctcctccctctcttctctctccctctctctctccccgtctctgtctctctcttttctctctctctctcacacacacctccctgactcctcactgaaaagc

SEQ ID NO: 19069 - RNA, 6140 nt, Homo sapiens
  source 1..6140: mol_type = other RNA
tgggagagaggactgtgaggcttcaccaataaacctccctagagttcagctaccaatgaggttaataccgctactaaataacatgaacatctgcaaaagattcagagatataatgatgtttgcactcagctttgcatcgaataaataatgccatttctatgttaaatccttcccttgtcaccatagatcttccaatcaaacaaagagtataccatctaccaacataggtccttagtccttcgtaaactactatgttaattcaggttcttaagatttagtcaggcatttgcagaaacatcaatatggatatagtgctatgagaaaagagaggcaggttttataagaagagttaacaaggaaaatatagaaaataagatgatagtaatgctaaatttacatatttcccgattcttctggtgtagacaaactaagaaatccaatagttacttgggaggcacttgaaggtgtgagtatgtataatagagtgcctttattgtatgattggcttgcagaattcaaagatagttccttgtatgcatggtctcaagattaattattgtaacagttccataaggttattgatcattctttgatctcctagtgtataatacaccctaatcagaatgtaccattcagcaagttggattgattcttggtaatttttgagaaattcaccccatcgtttcagacgagaagtgtctggaatgacaaattcacagtagatcatttaatatgctatctccccttagagtgtgcattgtttaattattgattgtgtagatcactgatggttgcagctcatatttcaaaaagtatgtactggaagtctatgcacagcaaaatgtacacctaaaggggtatatgtttcagaatgggaaatggggctctatacttcaatttgtctcttttttggtaatatataagatgattcgtgaagtataatcattgaagatcaaggcgaagtttgtgataaacttcagaaaaacagaaatgtaaaccaataaaggactgatctaggtttgggcaaaatagtctcataagtatatttcatttgaggtattacagttgtaaattaaataataattttttgctgtgttaagaattttttttaatatatcaacagtttagttgaaaacattttacattctttgggaaactggcattactcagggtcttaagtactgtcaccatcaaacaatggtagcaaattaattggaaaactttttttaaaaggaaagacattacatactaacaaccactgcactttctgagtcttgttaaatacaacttgtatgttcagagttgaagtctgagactcaaaaccaaatgtattcaacattattaagaagagacaaatagaataatgagcaatacaaacaaagcaaagacagcaaaacatttttcaagactattgatgtattgtattgaatataatacagagaaaggcaaaggggctttattatgcttgtggccactgaagatgcaaacaccggccacacaggatctgagaagcatttccaggtctatgaataacaccacgaggagacaaaagcaaacacagcaaatgttctcaaataaagcaaggacattatagtccaaatttaatttttacctctaacaaaacttatgtattacatggttaagagaccaaggctacagttttcacatgtaaaaactgtagccattaagcaggttaaacttgttttagatcataccagaacagttgaaaattaacagcaatatctaatttcttgttccatagaatgaatgctatgagaaatatatcactggacgaggcttcctggagccaccccaagcctgtacatggcaagatggcagtgctgcaagcccactgcctgtacattcagtgtaagagcattcgtttttccattgagaacccctggctattaaaacaaactatcataattttatgttaaatcatagctgccaatcagaagaagtactctttctgattttcattgactgcattttgtatattaagctcacttttcagaacagcctcagcactgtctacattctctgacctttttgcctcacttcttttatataaccttttctgctgataaatgcgaacagctatggcagtgatgcaaagcaagataaaaatcacaacagctatcagacctccaattactgcagagtcacttttgattgcattagcaaggggctctctgtcatctattgttccagaatgatctgcaaacgagtgtgtcctttcccttgatgtggcatcagtgccaggctgggccatacagctggactcagtcacgtgtcctgtaacagtgacagggtctgggtggctggggtgcagagctgccttcagaggggccacgtggctgagctgcactgcagagaggcagcctgtgaagccctgcgcacctgccagtgcagtatcctggtccacatcactgtgttctaaaatcctgcccaataccagagatttgactgcactgaattctgtgcctgatgacaggtgaacttgtctccttctattatcgtcaatctctataaagaccactccttcttctctgttaatcattatgtggtgaagttgtccatcagccatgtttttaaaatcaaagttaacaacatcaggctcttgatatttatttaacttgtacctgatctgcaaacttccatttttggcaatgatcacagaaaggtattctttgtaaaaggagctcacaaaaagcagcaagcttggtgttcgtgttgttcggaaactaaatttgatcatttctctgctcagcttcatatcaccatgaaatgaagcagcgtgggagctggagtttttacttaaaagataattttcttgaaaattgtatatcacggatgagccagatccaaaatatgcagaaatctcatttgagcagaatggccctgtgtatgcagagaaagtgcagtcacaaaagaacccaatgggtctttctctgcatttccctccattgcggcataacttcccatagctgctgcaatgtcccctacaacctggctgcacttctggagtcacctgggctctttcttccaaatccagggtcatcccattcaactgcagagaccgaatgcagcccagaaagcctctctgtctggtggccgttccacccacgaagagctgactgttgagctgtaacaggacatgcccatcagcgggggcgggctgtgtctttggtgtcagctgatccacttgaagggaggcctccttcatgttcctttcaaccctcacatggtgccactggttgtcgttgaagtgggtgggtgactgcactgagatttcaaaaggcccattccccacatcaaatgaaaaagtcactactgtcggagagcgaagctctatccgtataaaatcagcaatccccaagttctctaaaaataccccagatgaagctgttgtcttaaaaaagaaagatacatccgcgctaagttctccgtggaaggtaggaaaatgaagatatgaagcctcggtatcaaaggaagctgaattccaaaatgatctgtctccctggcagagcagaggccccagtttataagctgcttctgaatgcagtcggcctgtgtctgtaatcacgatcttagttactggaagatgttctttataagcaagcaatccagtgtcattggtccattcattccggtcagcatcacaattgcagtaatactgagaatcaatgcagtttccctctaatccacaagtacatttttgaagatcaggcgaagaacctccccagtaggtttgcgtttcattggttcttcctacccaccaactcagaggggttccatcttgcttattgaccagccgtgacttcttgcagtaataagtaaactcctgttcacagtgctctgcacggttaatagtggcctgaagttgctccatgctggccacatactcgaaaaacccagcatatgggttctctggattagtatttctgactcttgttaagtcagagccgttgtgctgtatgatggtccatgcagtttcggtcatattgcaatatagaagaaatggttccaggggaccacttccatctgaatctatatagtaaaaccctgaagtatttcctctgtgcttataggcttcacatgactgctcatagatagagttatggcaagtagctcctctgtaaccagtgttggtacagttacaatgaaaggtgctccaggactgggaacactccccaccgtgttcacaatagttgggcaaacacctgtctgagatgccacatgagtctatctgaaggtcactgaagttcccaagggacccctgctgaactgaaatcagatctaccactttgccgctgatagaaatgagcctcatacatccctgaaatccaccaagtggacttttacatttggatccaaagcttttgtcaggacaacctccaaaataataggtgccacccgaataaatctgctcaggccccagcagaggagcagcagaagccatctggccgtccaccgccacactcaagtgattctttttagcagataaagagacagaatgccactgcccatcatttaattcgacacctgctgtgatgtcactgggtaattttcctggctggtagagattcgacttaagttttccatcactcagaaagaggaggataccccctgaaatcagctgaagttcactgaacagcagaagccctgccttattccaagttcgaaattgaaaagtggcagaaacctcctcctctccagagaagtctggcagtgctaaataactcctggagctcagaaaagtcacgggcatagattgtggttgtgaacaagaaaatgacacatttcccatagcaatgatctgtggtttttgctgcttggccaaatcaatgatatccactccattataatagagattttctaaacatccatgaaaatttctatgtgggaatgacactgattttccaggtgctggaatccctccaaagctgatctcataatcaagattcatgagattgaattctccccgtgcatggaaatgatgcctgtgttcgtccactgtgaagttgacttgtttgcccaaacgctggatgagcactgaatgccaatgctgatcatctagcaggctgcccagggtgagattgaccagggtggaagtggaaggcagtttagcttcacctgaattaataagtaaaaagagtcttgctcttcttaattgcagtgtgatgtgatctccatttggcccttccctgtggagtagaatcccatcactctgcatggttttgaatttcaaagaaataatgtcttttattgggctcagggatttttgatcaaatctgtagagaagggaactttttccatcaagatcaaccacttctgatctgtatgcacatccgaacacttcgattcgcattccaattctgcccttggggttccattccaaagggatgaagcgcagaaatctggctttgatagaaggctggagtctatagtacacaacactgtctgcatttgcatttcctgaaaaaccccagatgctgtcctcttggcgatattgtttccagttccagccactatcactgaacatcaggaggtagctggtcacccagttggagctaccatatcccccttgagtggccacagcggtgacctccattctctctccaaggtcaatctgcaaccactggtatttgttagacacaagtggagaccagccaccagctccatctcttctattcagccttgcaaatccaggaccatgactgctggagagctcggaagaactgctgaaggatgcctgaggcaaggcagacacaagaggatcatcacagtcataggaattcccagcttcgactctgttccaattttgagtagataacagaagtagcgtcttgaggacagctcccgtgacagatcccatgttcacatttattgggctcccccaaaagatcttgagaggctctcagagcgctccagtcctcttctcagtagctctgccagctctgtctgggtcttcagcccctctaggtctctgtctctccccctcccttcctcctcacctccctccgtcttttcttcttccctcctccctctcttctctctccctctctctctccccgtctctgtctctctcttttctctctctctctcacacacacctccctgactcctcactgaaaagc

SEQ ID NO: 19070 - RNA, 5862 nt, Homo sapiens
  source 1..5862: mol_type = other RNA
tgggagagaggactgtgaggcttcaccaataaacctccctagagttcagctaccaatgaggttaataccgctactaaataacatgaacatctgcaaaagattcagagatataatgatgtttgcactcagctttgcatcgaataaataatgccatttctatgttaaatccttcccttgtcaccatagatcttccaatcaaacaaagagtataccatctaccaacataggtccttagtccttcgtaaactactatgttaattcaggttcttaagatttagtcaggcatttgcagaaacatcaatatggatatagtgctatgagaaaagagaggcaggttttataagaagagttaacaaggaaaatatagaaaataagatgatagtaatgctaaatttacatatttcccgattcttctggtgtagacaaactaagaaatccaatagttacttgggaggcacttgaaggtgtgagtatgtataatagagtgcctttattgtatgattggcttgcagaattcaaagatagttccttgtatgcatggtctcaagattaattattgtaacagttccataaggttattgatcattctttgatctcctagtgtataatacaccctaatcagaatgtaccattcagcaagttggattgattcttggtaatttttgagaaattcaccccatcgtttcagacgagaagtgtctggaatgacaaattcacagtagatcatttaatatgctatctccccttagagtgtgcattgtttaattattgattgtgtagatcactgatggttgcagctcatatttcaaaaagtatgtactggaagtctatgcacagcaaaatgtacacctaaaggggtatatgtttcagaatgggaaatggggctctatacttcaatttgtctcttttttggtaatatataagatgattcgtgaagtataatcattgaagatcaaggcgaagtttgtgataaacttcagaaaaacagaaatgtaaaccaataaaggactgatctaggtttgggcaaaatagtctcataagtatatttcatttgaggtattacagttgtaaattaaataataattttttgctgtgttaagaattttttttaatatatcaacagtttagttgaaaacattttacattctttgggaaactggcattactcagggtcttaagtactgtcaccatcaaacaatggtagcaaattaattggaaaactttttttaaaaggaaagacattacatactaacaaccactgcactttctgagtcttgttaaatacaacttgtatgttcagagttgaagtctgagactcaaaaccaaatgtattcaacattattaagaagagacaaatagaataatgagcaatacaaacaaagcaaagacagcaaaacatttttcaagactattgatgtattgtattgaatataatacagagaaaggcaaaggggctttattatgcttgtggccactgaagatgcaaacaccggccacacaggatctgagaagcatttccaggtctatgaataacaccacgaggagacaaaagcaaacacagcaaatgttctcaaataaagcaaggacattatagtccaaatttaatttttacctctaacaaaacttatgtattacatggttaagagaccaaggctacagttttcacatgtaaaaactgtagccattaagcaggttaaacttgttttagatcataccagaacagttgaaaattaacagcaatatctaatttcttgttccatagaatgaatgctatgagaaatatatcactggacgaggcttcctggagccaccccaagcctgtacatggcaagatggcagtgctgcaagcccactgcctgtacattcagtgtaagagcattcgtttttccattgagaacccctggctattaaaacaaactatcataattttatgttaaatcatagctgccaatcagaagaagtactctttctgattttcattgactgcattttgtatattaagctcacttttcagaacagcctcagcactgtctacattctctgacctttttgcctcacttcttttatataaccttttctgctgataaatgcgaacagctatggcagtgatgcaaagcaagataaaaatcacaacagctatcagacctccaattactgcagagtcacttttgattgcattagcaaggggctctctgtcatctattgttccagaatgatctgcaaacgagtgtgtcctttcccttgatgtggcatcagtgccaggctgggccatacagctggactcagtcacgtgtcctgtaacagtgacagggtctgggtggctggggtgcagagctgccttcagaggggccacgtggctgagctgcactgcagagaggcagcctgtgaagccctgcgcacctgccagtgcagtatcctggtccacatcactgtgttctaaaatcctgcccaataccagagatttgactgcactgaattctgtgcctgatgacaggtgaacttgtctccttctattatcgtcaatctctataaagaccactccttcttctctgttaatcattatgtggtgaagttgtccatcagccatgtttttaaaatcaaagttaacaacatcaggctcttgatatttatttaacttgtacctgatctgcaaacttccatttttggcaatgatcacagaaaggtattctttgtaaaaggagctcacaaaaagcagcaagcttggtgttcgtgttgttcggaaactaaatttgatcatttctctgctcagcttcatatcaccatgaaatgaagcagcgtgggagctggagtttttacttaaaagataattttcttgaaaattgtatatcacggatgagccagatccaaaatatgcagaaatctcatttgagcagaatggccctgtgtatgcagagaaagtgcagtcacaaaagaacccaatgggtctttctctgcatttccctccattgcggcataacttcccatagctgctgcaatgtcccctacaacctggctgcacttctggagtcacctgggctctttcttccaaatccagggtcatcccattcaactgcagagaccgaatgcagcccagaaagcctctctgtctggtggccgttccacccacgaagagctgactgttgagctgtaacaggacatgcccatcagcgggggcgggctgtgtctttggtgtcagctgatccacttgaagggaggcctccttcatgttcctttcaaccctcacatggtgccactggttgtcgttgaagtgggtgggtgactgcactgagatttcaaaaggcccattccccacatcaaatgaaaaagtcactactgtcggagagcgaagctctatccgtataaaatcagcaatccccaagttctctaaaaataccccagatgaagctgttgtcttaaaaaagaaagatacatccgcgctaagttctccgtggaaggtaggaaaatgaagatatgaagcctcggtatcaaaggaagctgaattccaaaatgatctgtctccctggcagagcagaggccccagtttataagctgcttctgaatgcagtcggcctgtgtctgtaatcacgatcttagttactggaagatgttctttataagcaagcaatccagtgtcattggtccattcattccggtcagcatcacaattgcagtaatactgagaatcaatgcagtttccctctaatccacaagtacatttttgaagatcaggcgaagaacctccccagtaggtttgcgtttcattggttcttcctacccaccaactcagaggggttccatcttgcttattgaccagccgtgacttcttgcagtaataagtaaactcctgttcacagtgctctgcacggttaatagtggcctgaagttgctccatgctggccacatactcgaaaaacccagcatatgggttctctggattagtatttctgactcttgttaagtcagagccgttgtgctgtatgatggtccatgcagtttcggtcatattgcaatatagaagaaatggttccaggggaccacttccatctgaatctatatagtaaaaccctgaagtatttcctctgtgcttataggcttcacatgactgctcatagatagagttatggcaagtagctcctctgtaaccagtgttggtacagttacaatgaaaggtgctccaggactgggaacactccccaccgtgttcacaatagttgggcaaacacctgtctgagatgccacatgagtctatctgaaggtcactgaagttcccaagggacccctgctgaactgaaatcagatctaccactttgccgctgatagaaatgagcctcatacatccctgaaatccaccaagtggacttttacatttggatccaaagcttttgtcaggacaacctccaaaataataggtgccacccgaataaatctgctcaggccccagcagaggagcagcagaagccatctggccgtccaccgccacactcaagtgattctttttagcagataaagagacagaatgccactgcccatcatttaattcgacacctgctgtgatgtcactgggtaattttcctggctggtagagattcgacttaagttttccatcactcagaaagaggaggataccccctgaaatcagctgaagttcactgaacagcagaagccctgccttattccaagttcgaaattgaaaagtggcagaaacctcctcctctccagagaagtctggcagtgctaaataactcctggagctcagaaaagtcacgggcatagattgtggttgtgaacaagaaaatgacacatttcccatagcaatgatctgtggtttttgctgcttggccaaatcaatgatatccactccattataatagagattttctaaacatccatgaaaatttctatgtgggaatgacactgattttccaggtgctggaatccctccaaagctgatctcataatcaagattcatgagattgaattctccccgtgcatggaaatgatgcctgtgttcgtccactgtgaagttgacttgtttgcccaaacgctggatgagcactgaatgccaatgctgatcatctagcaggctgcccagggtgagattgaccagggtggaagtggaaggcagtttagcttcacctgaattaataagtaaaaagagtcttgctcttcttaattgcagtgtgatgtgatctccatttggcccttccctgtggagtagaatcccatcactctgcatggttttgaatttcaaagaaataatgtcttttattgggctcagggatttttgatcaaatctgtagagaagggaactttttccatcaagatcaaccacttctgatctgtatgcacatccgaacacttcgattcgcattccaattctgcccttggggttccattccaaagggatgaagcgcagaaatctggctttgatagaaggctggagtctatagtacacaacactgtctgcatttgcatttcctgaaaaaccccagatgctgtcctcttggcgatattgtttccagttccagccactatcactgaacatcaggaggtagctggtcacccagttggagctaccatatcccccttgagtggccacagcggtgacctccattctctctccaaggtcaatctgcaaccactggtatttgttagacacaagtggagaccagccaccagctccatctcttctattcagccttgcaaatccaggaccatgactgctggagagctcggaagaactgctgaaggatgcctgaggcaaggcagacacaagaggatcatcacagtcatagttccacatagctgggaaggcctcagaatcatggcggctgcaagagaaaatgaggaagcagcaaaagc

SEQ ID NO: 19071 - RNA, 6399 nt, Homo sapiens
  source 1..6399: mol_type = other RNA
tgggagagaggactgtgaggcttcaccaataaacctccctagagttcagctaccaatgaggttaataccgctactaaataacatgaacatctgcaaaagattcagagatataatgatgtttgcactcagctttgcatcgaataaataatgccatttctatgttaaatccttcccttgtcaccatagatcttccaatcaaacaaagagtataccatctaccaacataggtccttagtccttcgtaaactactatgttaattcaggttcttaagatttagtcaggcatttgcagaaacatcaatatggatatagtgctatgagaaaagagaggcaggttttataagaagagttaacaaggaaaatatagaaaataagatgatagtaatgctaaatttacatatttcccgattcttctggtgtagacaaactaagaaatccaatagttacttgggaggcacttgaaggtgtgagtatgtataatagagtgcctttattgtatgattggcttgcagaattcaaagatagttccttgtatgcatggtctcaagattaattattgtaacagttccataaggttattgatcattctttgatctcctagtgtataatacaccctaatcagaatgtaccattcagcaagttggattgattcttggtaatttttgagaaattcaccccatcgtttcagacgagaagtgtctggaatgacaaattcacagtagatcatttaatatgctatctccccttagagtgtgcattgtttaattattgattgtgtagatcactgatggttgcagctcatatttcaaaaagtatgtactggaagtctatgcacagcaaaatgtacacctaaaggggtatatgtttcagaatgggaaatggggctctatacttcaatttgtctcttttttggtaatatataagatgattcgtgaagtataatcattgaagatcaaggcgaagtttgtgataaacttcagaaaaacagaaatgtaaaccaataaaggactgatctaggtttgggcaaaatagtctcataagtatatttcatttgaggtattacagttgtaaattaaataataattttttgctgtgttaagaattttttttaatatatcaacagtttagttgaaaacattttacattctttgggaaactggcattactcagggtcttaagtactgtcaccatcaaacaatggtagcaaattaattggaaaactttttttaaaaggaaagacattacatactaacaaccactgcactttctgagtcttgttaaatacaacttgtatgttcagagttgaagtctgagactcaaaaccaaatgtattcaacattattaagaagagacaaatagaataatgagcaatacaaacaaagcaaagacagcaaaacatttttcaagactattgatgtattgtattgaatataatacagagaaaggcaaaggggctttattatgcttgtggccactgaagatgcaaacaccggccacacaggatctgagaagcatttccaggtctatgaataacaccacgaggagacaaaagcaaacacagcaaatgttctcaaataaagcaaggacattatagtccaaatttaatttttacctctaacaaaacttatgtattacatggttaagagaccaaggctacagttttcacatgtaaaaactgtagccattaagcaggttaaacttgttttagatcataccagaacagttgaaaattaacagcaatatctaatttcttgttccatagaatgaatgctatgagaaatatatcactggacgaggcttcctggagccaccccaagcctgtacatggcaagatggcagtgctgcaagcccactgcctgtacattcagtgtaagagcattcgtttttccattgagaacccctggctattaaaacaaactatcataattttatgttaaatcatagctgccaatcagaagaagtactctttctgattttcattgactgcattttgtatattaagctcacttttcagaacagcctcagcactgtctacattctctgacctttttgcctcacttcttttatataaccttttctgctgataaatgcgaacagctatggcagtgatgcaaagcaagataaaaatcacaacagctatcagacctccaattactgcagagtcacttttgattgcattagcaaggggctctctgtcatctattgttccagaatgatctgcaaacgagtgtgtcctttcccttgatgtggcatcagtgccaggctgggccatacagctggactcagtcacgtgtcctgtaacagtgacagggtctgggtggctggggtgcagagctgccttcagaggggccacgtggctgagctgcactgcagagaggcagcctgtgaagccctgcgcacctgccagtgcagtatcctggtccacatcactgtgttctaaaatcctgcccaataccagagatttgactgcactgaattctgtgcctgatgacaggtgaacttgtctccttctattatcgtcaatctctataaagaccactccttcttctctgttaatcattatgtggtgaagttgtccatcagccatgtttttaaaatcaaagttaacaacatcaggctcttgatatttatttaacttgtacctgatctgcaaacttccatttttggcaatgatcacagaaaggtattctttgtaaaaggagctcacaaaaagcagcaagcttggtgttcgtgttgttcggaaactaaatttgatcatttctctgctcagcttcatatcaccatgaaatgaagcagcgtgggagctggagtttttacttaaaagataattttcttgaaaattgtatatcacggatgagccagatccaaaatatgcagaaatctcatttgagcagaatggccctgtgtatgcagagaaagtgcagtcacaaaagaacccaatgggtctttctctgcatttccctccattgcggcataacttcccatagctgctgcaatgtcccctacaacctggctgcacttctggagtcacctgggctctttcttccaaatccagggtcatcccattcaactgcagagaccgaatgcagcccagaaagcctctctgtctggtggccgttccacccacgaagagctgactgttgagctgtaacaggacatgcccatcagcgggggcgggctgtgtctttggtgtcagctgatccacttgaagggaggcctccttcatgttcctttcaaccctcacatggtgccactggttgtcgttgaagtgggtgggtgactgcactgagatttcaaaaggcccattccccacatcaaatgaaaaagtcactactgtcggagagcgaagctctatccgtataaaatcagcaatccccaagttctctaaaaataccccagatgaagctgttgtcttaaaaaagaaagatacatccgcgctaagttctccgtggaaggtaggaaaatgaagatatgaagcctcggtatcaaaggaagctgaattccaaaatgatctgtctccctggcagagcagaggccccagtttataagctgcttctgaatgcagtcggcctgtgtctgtaatcacgatcttagttactggaagatgttctttataagcaagcaatccagtgtcattggtccattcattccggtcagcatcacaattgcagtaatactgagaatcaatgcagtttccctctaatccacaagtacatttttgaagatcaggcgaagaacctccccagtaggtttgcgtttcattggttcttcctacccaccaactcagaggggttccatcttgcttattgaccagccgtgacttcttgcagtaataagtaaactcctgttcacagtgctctgcacggttaatagtggcctgaagttgctccatgctggccacatactcgaaaaacccagcatatgggttctctggattagtatttctgactcttgttaagtcagagccgttgtgctgtatgatggtccatgcagtttcggtcatattgcaatatagaagaaatggttccaggggaccacttccatctgaatctatatagtaaaaccctgaagtatttcctctgtgcttataggcttcacatgactgctcatagatagagttatggcaagtagctcctctgtaaccagtgttggtacagttacaatgaaaggtgctccaggactgggaacactccccaccgtgttcacaatagttgggcaaacacctgtctgagatgccacatgagtctatctgaaggtcactgaagttcccaagggacccctgctgaactgaaatcagatctaccactttgccgctgatagaaatgagcctcatacatccctgaaatccaccaagtggacttttacatttggatccaaagcttttgtcaggacaacctccaaaataataggtgccacccgaataaatctgctcaggccccagcagaggagcagcagaagccatctggccgtccaccgccacactcaagtgattctttttagcagataaagagacagaatgccactgcccatcatttaattcgacacctgctgtgatgtcactgggtaattttcctggctggtagagattcgacttaagttttccatcactcagaaagaggaggataccccctgaaatcagctgaagttcactgaacagcagaagccctgccttattccaagttcgaaattgaaaagtggcagaaacctcctcctctccagagaagtctggcagtgctaaataactcctggagctcagaaaagtcacgggcatagattgtggttgtgaacaagaaaatgacacatttcccatagcaatgatctgtggtttttgctgcttggccaaatcaatgatatccactccattataatagagattttctaaacatccatgaaaatttctatgtgggaatgacactgattttccaggtgctggaatccctccaaagctgatctcataatcaagattcatgagattgaattctccccgtgcatggaaatgatgcctgtgttcgtccactgtgaagttgacttgtttgcccaaacgctggatgagcactgaatgccaatgctgatcatctagcaggctgcccagggtgagattgaccagggtggaagtggaaggcagtttagcttcacctgaattaataagtaaaaagagtcttgctcttcttaattgcagtgtgatgtgatctccatttggcccttccctgtggagtagaatcccatcactctgcatggttttgaatttcaaagaaataatgtcttttattgggctcagggatttttgatcaaatctgtagagaagggaactttttccatcaagatcaaccacttctgatctgtatgcacatccgaacacttcgattcgcattccaattctgcccttggggttccattccaaagggatgaagcgcagaaatctggctttgatagaaggctggagtctatagtacacaacactgtctgcatttgcatttcctgaaaaaccccagatgctgtcctcttggcgatattgtttccagttccagccactatcactgaacatcaggaggtagctggtcacccagttggagctaccatatcccccttgagtggccacagcggtgacctccattctctctccaaggtcaatctgcaaccactggtatttgttagacacaagtggagaccagccaccagctccatctcttctattcagccttgcaaatccaggaccatgactgctggagagctcggaagaactgctgaaggatgcctgaggcaaggcagacacaagaggatcatcacagtcatcatggcatattcctcaaacattgcattgtagaaatcacacacaatctcaaaaaagcttttaaatacgatcctttgtagagaagtttaggaagagagtttcaaaaaatgaacacacttaaaatttcttattcagtagctggccatggtggcacatgtctgtaatctccgctagtctacttgggaggctgaggcaggagaatcgctggaacccaggaggcagaggctgcagtgagctgagattgcaccactacattccagcaggaattcccagcttcgactctgttccaattttgagtagataacagaagtagcgtcttgaggacagctcccgtgacagatcccatgttcacatttattgggctcccccaaaagatcttgagaggctctcagagcgctccagtcctcttctcagtagctctgccagctctgtctgggtcttcagcccctctaggtctctgtctctccccctcccttcctcctcacctccctccgtcttttcttcttccctcctccctctcttctctctccctctctctctccccgtctctgtctctctcttttctctctctctctcacacacacctccctgactcctcactgaaaagc

SEQ ID NO: 19072 - RNA, 5996 nt, Homo sapiens
  source 1..5996: mol_type = other RNA
tgggagagaggactgtgaggcttcaccaataaacctccctagagttcagctaccaatgaggttaataccgctactaaataacatgaacatctgcaaaagattcagagatataatgatgtttgcactcagctttgcatcgaataaataatgccatttctatgttaaatccttcccttgtcaccatagatcttccaatcaaacaaagagtataccatctaccaacataggtccttagtccttcgtaaactactatgttaattcaggttcttaagatttagtcaggcatttgcagaaacatcaatatggatatagtgctatgagaaaagagaggcaggttttataagaagagttaacaaggaaaatatagaaaataagatgatagtaatgctaaatttacatatttcccgattcttctggtgtagacaaactaagaaatccaatagttacttgggaggcacttgaaggtgtgagtatgtataatagagtgcctttattgtatgattggcttgcagaattcaaagatagttccttgtatgcatggtctcaagattaattattgtaacagttccataaggttattgatcattctttgatctcctagtgtataatacaccctaatcagaatgtaccattcagcaagttggattgattcttggtaatttttgagaaattcaccccatcgtttcagacgagaagtgtctggaatgacaaattcacagtagatcatttaatatgctatctccccttagagtgtgcattgtttaattattgattgtgtagatcactgatggttgcagctcatatttcaaaaagtatgtactggaagtctatgcacagcaaaatgtacacctaaaggggtatatgtttcagaatgggaaatggggctctatacttcaatttgtctcttttttggtaatatataagatgattcgtgaagtataatcattgaagatcaaggcgaagtttgtgataaacttcagaaaaacagaaatgtaaaccaataaaggactgatctaggtttgggcaaaatagtctcataagtatatttcatttgaggtattacagttgtaaattaaataataattttttgctgtgttaagaattttttttaatatatcaacagtttagttgaaaacattttacattctttgggaaactggcattactcagggtcttaagtactgtcaccatcaaacaatggtagcaaattaattggaaaactttttttaaaaggaaagacattacatactaacaaccactgcactttctgagtcttgttaaatacaacttgtatgttcagagttgaagtctgagactcaaaaccaaatgtattcaacattattaagaagagacaaatagaataatgagcaatacaaacaaagcaaagacagcaaaacatttttcaagactattgatgtattgtattgaatataatacagagaaaggcaaaggggctttattatgcttgtggccactgaagatgcaaacaccggccacacaggatctgagaagcatttccaggtctatgaataacaccacgaggagacaaaagcaaacacagcaaatgttctcaaataaagcaaggacattatagtccaaatttaatttttacctctaacaaaacttatgtattacatggttaagagaccaaggctacagttttcacatgtaaaaactgtagccattaagcaggttaaacttgttttagatcataccagaacagttgaaaattaacagcaatatctaatttcttgttccatagaatgaatgctatgagaaatatatcactggacgaggcttcctggagccaccccaagcctgtacatggcaagatggcagtgctgcaagcccactgcctgtacattcagtgtaagagcattcgtttttccattgagaacccctggctattaaaacaaactatcataattttatgttaaatcatagctgccaatcagaagaagtactctttctgattttcattgactgcattttgtatattaagctcacttttcagaacagcctcagcactgtctacattctctgacctttttgcctcacttcttttatataaccttttctgctgataaatgcgaacagctatggcagtgatgcaaagcaagataaaaatcacaacagctatcagacctccaattactgcagagtcacttttgattgcattagcaaggggctctctgtcatctattgttccagaatgatctgcaaacgagtgtgtcctttcccttgatgtggcatcagtgccaggctgggccatacagctggactcagtcacgtgtcctgtaacagtgacagggtctgggtggctggggtgcagagctgccttcagaggggccacgtggctgagctgcactgcagagaggcagcctgtgaagccctgcgcacctgccagtgcagtatcctggtccacatcactgtgttctaaaatcctgcccaataccagagatttgactgcactgaattctgtgcctgatgacaggtgaacttgtctccttctattatcgtcaatctctataaagaccactccttcttctctgttaatcattatgtggtgaagttgtccatcagccatgtttttaaaatcaaagttaacaacatcaggctcttgatatttatttaacttgtacctgatctgcaaacttccatttttggcaatgatcacagaaaggtattctttgtaaaaggagctcacaaaaagcagcaagcttggtgttcgtgttgttcggaaactaaatttgatcatttctctgctcagcttcatatcaccatgaaatgaagcagcgtgggagctggagtttttacttaaaagataattttcttgaaaattgtatatcacggatgagccagatccaaaatatgcagaaatctcatttgagcagaatggccctgtgtatgcagagaaagtgcagtcacaaaagaacccaatgggtctttctctgcatttccctccattgcggcataacttcccatagctgctgcaatgtcccctacaacctggctgcacttctggagtcacctgggctctttcttccaaatccagggtcatcccattcaactgcagagaccgaatgcagcccagaaagcctctctgtctggtggccgttccacccacgaagagctgactgttgagctgtaacaggacatgcccatcagcgggggcgggctgtgtctttggtgtcagctgatccacttgaagggaggcctccttcatgttcctttcaaccctcacatggtgccactggttgtcgttgaagtgggtgggtgactgcactgagatttcaaaaggcccattccccacatcaaatgaaaaagtcactactgtcggagagcgaagctctatccgtataaaatcagcaatccccaagttctctaaaaataccccagatgaagctgttgtcttaaaaaagaaagatacatccgcgctaagttctccgtggaaggtaggaaaatgaagatatgaagcctcggtatcaaaggaagctgaattccaaaatgatctgtctccctggcagagcagaggccccagtttataagctgcttctgaatgcagtcggcctgtgtctgtaatcacgatcttagttactggaagatgttctttataagcaagcaatccagtgtcattggtccattcattccggtcagcatcacaattgcagtaatactgagaatcaatgcagtttccctctaatccacaagtacatttttgaagatcaggcgaagaacctccccagtaggtttgcgtttcattggttcttcctacccaccaactcagaggggttccatcttgcttattgaccagccgtgacttcttgcagtaataagtaaactcctgttcacagtgctctgcacggttaatagtggcctgaagttgctccatgctggccacatactcgaaaaacccagcatatgggttctctggattagtatttctgactcttgttaagtcagagccgttgtgctgtatgatggtccatgcagtttcggtcatattgcaatatagaagaaatggttccaggggaccacttccatctgaatctatatagtaaaaccctgaagtatttcctctgtgcttataggcttcacatgactgctcatagatagagttatggcaagtagctcctctgtaaccagtgttggtacagttacaatgaaaggtgctccaggactgggaacactccccaccgtgttcacaatagttgggcaaacacctgtctgagatgccacatgagtctatctgaaggtcactgaagttcccaagggacccctgctgaactgaaatcagatctaccactttgccgctgatagaaatgagcctcatacatccctgaaatccaccaagtggacttttacatttggatccaaagcttttgtcaggacaacctccaaaataataggtgccacccgaataaatctgctcaggccccagcagaggagcagcagaagccatctggccgtccaccgccacactcaagtgattctttttagcagataaagagacagaatgccactgcccatcatttaattcgacacctgctgtgatgtcactgggtaattttcctggctggtagagattcgacttaagttttccatcactcagaaagaggaggataccccctgaaatcagctgaagttcactgaacagcagaagccctgccttattccaagttcgaaattgaaaagtggcagaaacctcctcctctccagagaagtctggcagtgctaaataactcctggagctcagaaaagtcacgggcatagattgtggttgtgaacaagaaaatgacacatttccctcataatcaagattcatgagattgaattctccccgtgcatggaaatgatgcctgtgttcgtccactgtgaagttgacttgtttgcccaaacgctggatgagcactgaatgccaatgctgatcatctagcaggctgcccagggtgagattgaccagggtggaagtggaaggcagtttagcttcacctgaattaataagtaaaaagagtcttgctcttcttaattgcagtgtgatgtgatctccatttggcccttccctgtggagtagaatcccatcactctgcatggttttgaatttcaaagaaataatgtcttttattgggctcagggatttttgatcaaatctgtagagaagggaactttttccatcaagatcaaccacttctgatctgtatgcacatccgaacacttcgattcgcattccaattctgcccttggggttccattccaaagggatgaagcgcagaaatctggctttgatagaaggctggagtctatagtacacaacactgtctgcatttgcatttcctgaaaaaccccagatgctgtcctcttggcgatattgtttccagttccagccactatcactgaacatcaggaggtagctggtcacccagttggagctaccatatcccccttgagtggccacagcggtgacctccattctctctccaaggtcaatctgcaaccactggtatttgttagacacaagtggagaccagccaccagctccatctcttctattcagccttgcaaatccaggaccatgactgctggagagctcggaagaactgctgaaggatgcctgaggcaaggcagacacaagaggatcatcacagtcataggaattcccagcttcgactctgttccaattttgagtagataacagaagtagcgtcttgaggacagctcccgtgacagatcccatgttcacatttattgggctcccccaaaagatcttgagaggctctcagagcgctccagtcctcttctcagtagctctgccagctctgtctgggtcttcagcccctctaggtctctgtctctccccctcccttcctcctcacctccctccgtcttttcttcttccctcctccctctcttctctctccctctctctctccccgtctctgtctctctcttttctctctctctctcacacacacctccctgactcctcactgaaaagc

SEQ ID NO: 19073 - RNA, 5704 nt, Homo sapiens
  source 1..5704: mol_type = other RNA
tgggagagaggactgtgaggcttcaccaataaacctccctagagttcagctaccaatgaggttaataccgctactaaataacatgaacatctgcaaaagattcagagatataatgatgtttgcactcagctttgcatcgaataaataatgccatttctatgttaaatccttcccttgtcaccatagatcttccaatcaaacaaagagtataccatctaccaacataggtccttagtccttcgtaaactactatgttaattcaggttcttaagatttagtcaggcatttgcagaaacatcaatatggatatagtgctatgagaaaagagaggcaggttttataagaagagttaacaaggaaaatatagaaaataagatgatagtaatgctaaatttacatatttcccgattcttctggtgtagacaaactaagaaatccaatagttacttgggaggcacttgaaggtgtgagtatgtataatagagtgcctttattgtatgattggcttgcagaattcaaagatagttccttgtatgcatggtctcaagattaattattgtaacagttccataaggttattgatcattctttgatctcctagtgtataatacaccctaatcagaatgtaccattcagcaagttggattgattcttggtaatttttgagaaattcaccccatcgtttcagacgagaagtgtctggaatgacaaattcacagtagatcatttaatatgctatctccccttagagtgtgcattgtttaattattgattgtgtagatcactgatggttgcagctcatatttcaaaaagtatgtactggaagtctatgcacagcaaaatgtacacctaaaggggtatatgtttcagaatgggaaatggggctctatacttcaatttgtctcttttttggtaatatataagatgattcgtgaagtataatcattgaagatcaaggcgaagtttgtgataaacttcagaaaaacagaaatgtaaaccaataaaggactgatctaggtttgggcaaaatagtctcataagtatatttcatttgaggtattacagttgtaaattaaataataattttttgctgtgttaagaattttttttaatatatcaacagtttagttgaaaacattttacattctttgggaaactggcattactcagggtcttaagtactgtcaccatcaaacaatggtagcaaattaattggaaaactttttttaaaaggaaagacattacatactaacaaccactgcactttctgagtcttgttaaatacaacttgtatgttcagagttgaagtctgagactcaaaaccaaatgtattcaacattattaagaagagacaaatagaataatgagcaatacaaacaaagcaaagacagcaaaacatttttcaagactattgatgtattgtattgaatataatacagagaaaggcaaaggggctttattatgcttgtggccactgaagatgcaaacaccggccacacaggatctgagaagcatttccaggtctatgaataacaccacgaggagacaaaagcaaacacagcaaatgttctcaaataaagcaaggacattatagtccaaatttaatttttacctctaacaaaacttatgtattacatggttaagagaccaaggctacagttttcacatgtaaaaactgtagccattaagcaggttaaacttgttttagatcataccagaacagttgaaaattaacagcaatatctaatttcttgttccatagaatgaatgctatgagaaatatatcactggacgaggcttcctggagccaccccaagcctgtacatggcaagatggcagtgctgcaagcccactgcctgtacattcagtgtaagagcattcgtttttccattgagaacccctggctattaaaacaaactatcataattttatgttaaatcatagctgccaatcagaagaagtactctttctgattttcattgactgcattttgtatattaagctcacttttcagaacagcctcagcactgtctacattctctgacctttttgcctcacttcttttatataaccttttctgctgataaatgcgaacagctatggcagtgatgcaaagcaagataaaaatcacaacagctatcagacctccaattactgcagagtcacttttgattgcattagcaaggggctctctgtcatctattgttccagaatgatctgcaaacgagtgtgtcctttcccttgatgtggcatcagtgccaggctgggccatacagctggactcagtcacgtgtcctgtaacagtgacagggtctgggtggctggggtgcagagctgccttcagaggggccacgtggctgagctgcactgcagagaggcagcctgtgaagccctgcgcacctgccagtgcagtatcctggtccacatcactgtgttctaaaatcctgcccaataccagagatttgactgcactgaattctgtgcctgatgacaggtgaacttgtctccttctattatcgtcaatctctataaagaccactccttcttctctgttaatcattatgtggtgaagttgtccatcagccatgtttttaaaatcaaagttaacaacatcaggctcttgatatttatttaacttgtacctgatctgcaaacttccatttttggcaatgatcacagaaaggtattctttgtaaaaggagctcacaaaaagcagcaagcttggtgttcgtgttgttcggaaactaaatttgatcatttctctgctcagcttcatatcaccatgaaatgaagcagcgtgggagctggagtttttacttaaaagataattttcttgaaaattgtatatcacggatgagccagatccaaaatatgcagaaatctcatttgagcagaatggccctgtgtatgcagagaaagtgcagtcacaaaagaacccaatgggtctttctctgcatttccctccattgcggcataacttcccatagctgctgcaatgtcccctacaacctggctgcacttctggagtcacctgggctctttcttccaaatccagggtcatcccattcaactgcagagaccgaatgcagcccagaaagcctctctgtctggtggccgttccacccacgaagagctgactgttgagctgtaacaggacatgcccatcagcgggggcgggctgtgtctttggtgtcagctgatccacttgaagggaggcctccttcatgttcctttcaaccctcacatggtgccactggttgtcgttgaagtgggtgggtgactgcactgagatttcaaaaggcccattccccacatcaaatgaaaaagtcactactgtcggagagcgaagctctatccgtataaaatcagcaatccccaagttctctaaaaataccccagatgaagctgttgtcttaaaaaagaaagatacatccgcgctaagttctccgtggaaggtaggaaaatgaagatatgaagcctcggtatcaaaggaagctgaattccaaaatgatctgtctccctggcagagcagaggccccagtttataagctgcttctgaatgcagtcggcctgtgtctgtaatcacgatcttagttactggaagatgttctttataagcaagcaatccagtgtcattggtccattcattccggtcagcatcacaattgcagtaatactgagaatcaatgcagtttccctctaatccacaagtacatttttgaagatcaggcgaagaacctccccagtaggtttgcgtttcattggttcttcctacccaccaactcagaggggttccatcttgcttattgaccagccgtgacttcttgcagtaataagtaaactcctgttcacagtgctctgcacggttaatagtggcctgaagttgctccatgctggccacatactcgaaaaacccagcatatgggttctctggattagtatttctgactcttgttaagtcagagccgttgtgctgtatgatggtccatgcagtttcggtcatattgcaatatagaagaaatggttccaggggaccacttccatctgaatctatatagtaaaaccctgaagtatttcctctgtgcttataggcttcacatgactgctcatagatagagttatggcaagtagctcctctgtaaccagtgttggtacagttacaatgaaaggtgctccaggactgggaacactccccaccgtgttcacaatagttgggcaaacacctgtctgagatgccacatgagtctatctgaaggtcactgaagttcccaagggacccctgctgaactgaaatcagatctaccactttgccgctgatagaaatgagcctcatacatccctgaaatccaccaagtggacttttacatttggatccaaagcttttgtcaggacaacctccaaaataataggtgccacccgaataaatctgctcaggccccagcagaggagcagcagaagccatctggccgtccaccgccacactcaagtgattctttttagcagataaagagacagaatgccactgcccatcatttaattcgacacctgctgtgatgtcactgggtaattttcctggctggtagagattcgacttaagttttccatcactcagaaagaggaggataccccctgaaatcagctgaagttcactgaacagcagaagccctgccttattccaagttcgaaattgaaaagtggcagaaacctcctcctctccagagaagtctggcagtgctaaataactcctggagctcagaaaagtcacgggcatagattgtggttgtgaacaagaaaatgacacatttccctcataatcaagattcatgagattgaattctccccgtgcatggaaatgatgcctgtgttcgtccactgtgaagttgacttgtttgcccaaacgctggatgagcactgaatgccaatgctgatcatctagcaggctgcccagggtgagattgaccagggtggaagtggaaggcagtttagcttcacctgaattaataagtaaaaagagtcttgctcttcttaattgcagtgtgatgtgatctccatttggcccttccctgtggagtagaatcccatcactctgcatggttttgaatttcaaagaaataatgtcttttattgggctcagggatttttgatcaaatctgtagagaagggaactttttccatcaagatcaaccacttctgatctgtatgcacatccgaacacttcgattcgcattccaattctgcccttggggttccattccaaagggatgaagcgcagaaatctggctttgatagaaggctggagtctatagtacacaacactgtctgcatttgcatttcctgaaaaaccccagatgctgtcctcttggcgatattgtttccagttccagccactatcactgaacatcaggaggtagctggtcacccagttggagctaccatatcccccttgagtggccacagcggtgacctccattctctctccaaggtcaatctgcaaccactggtatttgttagacacaagtggagaccagccaccagctccatctcttctattcagccttgcaaatccaggaccatgactgctggagagctcggaagaactgctgaaggatgcctgaggcaaggcagacacaagaggatcatcacagtcatagttccacatagctgggaaggcctcagaatcatggcggctgcaagagaaaatgag

SEQ ID NO: 19074 - RNA, 6205 nt, Homo sapiens
  source 1..6205: mol_type = other RNA
tgggagagaggactgtgaggcttcaccaataaacctccctagagttcagctaccaatgaggttaataccgctactaaataacatgaacatctgcaaaagattcagagatataatgatgtttgcactcagctttgcatcgaataaataatgccatttctatgttaaatccttcccttgtcaccatagatcttccaatcaaacaaagagtataccatctaccaacataggtccttagtccttcgtaaactactatgttaattcaggttcttaagatttagtcaggcatttgcagaaacatcaatatggatatagtgctatgagaaaagagaggcaggttttataagaagagttaacaaggaaaatatagaaaataagatgatagtaatgctaaatttacatatttcccgattcttctggtgtagacaaactaagaaatccaatagttacttgggaggcacttgaaggtgtgagtatgtataatagagtgcctttattgtatgattggcttgcagaattcaaagatagttccttgtatgcatggtctcaagattaattattgtaacagttccataaggttattgatcattctttgatctcctagtgtataatacaccctaatcagaatgtaccattcagcaagttggattgattcttggtaatttttgagaaattcaccccatcgtttcagacgagaagtgtctggaatgacaaattcacagtagatcatttaatatgctatctccccttagagtgtgcattgtttaattattgattgtgtagatcactgatggttgcagctcatatttcaaaaagtatgtactggaagtctatgcacagcaaaatgtacacctaaaggggtatatgtttcagaatgggaaatggggctctatacttcaatttgtctcttttttggtaatatataagatgattcgtgaagtataatcattgaagatcaaggcgaagtttgtgataaacttcagaaaaacagaaatgtaaaccaataaaggactgatctaggtttgggcaaaatagtctcataagtatatttcatttgaggtattacagttgtaaattaaataataattttttgctgtgttaagaattttttttaatatatcaacagtttagttgaaaacattttacattctttgggaaactggcattactcagggtcttaagtactgtcaccatcaaacaatggtagcaaattaattggaaaactttttttaaaaggaaagacattacatactaacaaccactgcactttctgagtcttgttaaatacaacttgtatgttcagagttgaagtctgagactcaaaaccaaatgtattcaacattattaagaagagacaaatagaataatgagcaatacaaacaaagcaaagacagcaaaacatttttcaagactattgatgtattgtattgaatataatacagagaaaggcaaaggggctttattatgcttgtggccactgaagatgcaaacaccggccacacaggatctgagaagcatttccaggtctatgaataacaccacgaggagacaaaagcaaacacagcaaatgttctcaaataaagcaaggacattatagtccaaatttaatttttacctctaacaaaacttatgtattacatggttaagagaccaaggctacagttttcacatgtaaaaactgtagccattaagcaggttaaacttgttttagatcataccagaacagttgaaaattaacagcaatatctaatttcttgttccatagaatgaatgctatgagaaatatatcactggacgaggcttcctggagccaccccaagcctgtacatggcaagatggcagtgctgcaagcccactgcctgtacattcagtgtaagagcattcgtttttccattgagaacccctggctattaaaacaaactatcataattttatgttaaatcatagctgccaatcagaagaagtactctttctgattttcattgactgcattttgtatattaagctcacttttcagaacagcctcagcactgtctacattctctgacctttttgcctcacttcttttatataaccttttctgctgataaatgcgaacagctatggcagtgatgcaaagcaagataaaaatcacaacagctatcagacctccaattactgcagagtcacttttgattgcattagcaaggggctctctgtcatctattgttccagaatgatctgcaaacgagtgtgtcctttcccttgatgtggcatcagtgccaggctgggccatacagctggactcagtcacgtgtcctgtaacagtgacagggtctgggtggctggggtgcagagctgccttcagaggggccacgtggctgagctgcactgcagagaggcagcctgtgaagccctgcgcacctgccagtgcagtatcctggtccacatcactgtgttctaaaatcctgcccaataccagagatttgactgcactgaattctgtgcctgatgacaggtgaacttgtctccttctattatcgtcaatctctataaagaccactccttcttctctgttaatcattatgtggtgaagttgtccatcagccatgtttttaaaatcaaagttaacaacatcaggctcttgatatttatttaacttgtacctgatctgcaaacttccatttttggcaatgatcacagaaaggtattctttgtaaaaggagctcacaaaaagcagcaagcttggtgttcgtgttgttcggaaactaaatttgatcatttctctgctcagcttcatatcaccatgaaatgaagcagcgtgggagctggagtttttacttaaaagataattttcttgaaaattgtatatcacggatgagccagatccaaaatatgcagaaatctcatttgagcagaatggccctgtgtatgcagagaaagtgcagtcacaaaagaacccaatgggtctttctctgcatttccctccattgcggcataacttcccatagctgctgcaatgtcccctacaacctggctgcacttctggagtcacctgggctctttcttccaaatccagggtcatcccattcaactgcagagaccgaatgcagcccagaaagcctctctgtctggtggccgttccacccacgaagagctgactgttgagctgtaacaggacatgcccatcagcgggggcgggctgtgtctttggtgtcagctgatccacttgaagggaggcctccttcatgttcctttcaaccctcacatggtgccactggttgtcgttgaagtgggtgggtgactgcactgagatttcaaaaggcccattccccacatcaaatgaaaaagtcactactgtcggagagcgaagctctatccgtataaaatcagcaatccccaagttctctaaaaataccccagatgaagctgttgtcttaaaaaagaaagatacatccgcgctaagttctccgtggaaggtaggaaaatgaagatatgaagcctcggtatcaaaggaagctgaattccaaaatgatctgtctccctggcagagcagaggccccagtttataagctgcttctgaatgcagtcggcctgtgtctgtaatcacgatcttagttactggaagatgttctttataagcaagcaatccagtgtcattggtccattcattccggtcagcatcacaattgcagtaatactgagaatcaatgcagtttccctctaatccacaagtacatttttgaagatcaggcgaagaacctccccagtaggtttgcgtttcattggttcttcctacccaccaactcagaggggttccatcttgcttattgaccagccgtgacttcttgcagtaataagtaaactcctgttcacagtgctctgcacggttaatagtggcctgaagttgctccatgctggccacatactcgaaaaacccagcatatgggttctctggattagtatttctgactcttgttaagtcagagccgttgtgctgtatgatggtccatgcagtttcggtcatattgcaatatagaagaaatggttccaggggaccacttccatctgaatctatatagtaaaaccctgaagtatttcctctgtgcttataggcttcacatgactgctcatagatagagttatggcaagtagctcctctgtaaccagtgttggtacagttacaatgaaaggtgctccaggactgggaacactccccaccgtgttcacaatagttgggcaaacacctgtctgagatgccacatgagtctatctgaaggtcactgaagttcccaagggacccctgctgaactgaaatcagatctaccactttgccgctgatagaaatgagcctcatacatccctgaaatccaccaagtggacttttacatttggatccaaagcttttgtcaggacaacctccaaaataataggtgccacccgaataaatctgctcaggccccagcagaggagcagcagaagccatctggccgtccaccgccacactcaagtgattctttttagcagataaagagacagaatgccactgcccatcatttaattcgacaccttaaatacggagaaaatgaggctcagagaggaaaagaaactaccgaggtcacatccagctgctggatagctgctgtgatgtcactgggtaattttcctggctggtagagattcgacttaagttttccatcactcagaaagaggaggataccccctgaaatcagctgaagttcactgaacagcagaagccctgccttattccaagttcgaaattgaaaagtggcagaaacctcctcctctccagagaagtctggcagtgctaaataactcctggagctcagaaaagtcacgggcatagattgtggttgtgaacaagaaaatgacacatttcccatagcaatgatctgtggtttttgctgcttggccaaatcaatgatatccactccattataatagagattttctaaacatccatgaaaatttctatgtgggaatgacactgattttccaggtgctggaatccctccaaagctcataatcaagattcatgagattgaattctccccgtgcatggaaatgatgcctgtgttcgtccactgtgaagttgacttgtttgcccaaacgctggatgagcactgaatgccaatgctgatcatctagcaggctgcccagggtgagattgaccagggtggaagtggaaggcagtttagcttcacctgaattaataagtaaaaagagtcttgctcttcttaattgcagtgtgatgtgatctccatttggcccttccctgtggagtagaatcccatcactctgcatggttttgaatttcaaagaaataatgtcttttattgggctcagggatttttgatcaaatctgtagagaagggaactttttccatcaagatcaaccacttctgatctgtatgcacatccgaacacttcgattcgcattccaattctgcccttggggttccattccaaagggatgaagcgcagaaatctggctttgatagaaggctggagtctatagtacacaacactgtctgcatttgcatttcctgaaaaaccccagatgctgtcctcttggcgatattgtttccagttccagccactatcactgaacatcaggaggtagctggtcacccagttggagctaccatatcccccttgagtggccacagcggtgacctccattctctctccaaggtcaatctgcaaccactggtatttgttagacacaagtggagaccagccaccagctccatctcttctattcagccttgcaaatccaggaccatgactgctggagagctcggaagaactgctgaaggatgcctgaggcaaggcagacacaagaggatcatcacagtcataggaattcccagcttcgactctgttccaattttgagtagataacagaagtagcgtcttgaggacagctcccgtgacagatcccatgttcacatttattgggctcccccaaaagatcttgagaggctctcagagcgctccagtcctcttctcagtagctctgccagctctgtctgggtcttcagcccctctaggtctctgtctctccccctcccttcctcctcacctccctccgtcttttcttcttccctcctccctctcttctctctccctctctctctccccgtctctgtctctctcttttctctctctctctcacacacacctccctgactcctcactgaaaagc

SEQ ID NO: 19075 - RNA, 5990 nt, Homo sapiens
  source 1..5990: mol_type = other RNA
tgggagagaggactgtgaggcttcaccaataaacctccctagagttcagctaccaatgaggttaataccgctactaaataacatgaacatctgcaaaagattcagagatataatgatgtttgcactcagctttgcatcgaataaataatgccatttctatgttaaatccttcccttgtcaccatagatcttccaatcaaacaaagagtataccatctaccaacataggtccttagtccttcgtaaactactatgttaattcaggttcttaagatttagtcaggcatttgcagaaacatcaatatggatatagtgctatgagaaaagagaggcaggttttataagaagagttaacaaggaaaatatagaaaataagatgatagtaatgctaaatttacatatttcccgattcttctggtgtagacaaactaagaaatccaatagttacttgggaggcacttgaaggtgtgagtatgtataatagagtgcctttattgtatgattggcttgcagaattcaaagatagttccttgtatgcatggtctcaagattaattattgtaacagttccataaggttattgatcattctttgatctcctagtgtataatacaccctaatcagaatgtaccattcagcaagttggattgattcttggtaatttttgagaaattcaccccatcgtttcagacgagaagtgtctggaatgacaaattcacagtagatcatttaatatgctatctccccttagagtgtgcattgtttaattattgattgtgtagatcactgatggttgcagctcatatttcaaaaagtatgtactggaagtctatgcacagcaaaatgtacacctaaaggggtatatgtttcagaatgggaaatggggctctatacttcaatttgtctcttttttggtaatatataagatgattcgtgaagtataatcattgaagatcaaggcgaagtttgtgataaacttcagaaaaacagaaatgtaaaccaataaaggactgatctaggtttgggcaaaatagtctcataagtatatttcatttgaggtattacagttgtaaattaaataataattttttgctgtgttaagaattttttttaatatatcaacagtttagttgaaaacattttacattctttgggaaactggcattactcagggtcttaagtactgtcaccatcaaacaatggtagcaaattaattggaaaactttttttaaaaggaaagacattacatactaacaaccactgcactttctgagtcttgttaaatacaacttgtatgttcagagttgaagtctgagactcaaaaccaaatgtattcaacattattaagaagagacaaatagaataatgagcaatacaaacaaagcaaagacagcaaaacatttttcaagactattgatgtattgtattgaatataatacagagaaaggcaaaggggctttattatgcttgtggccactgaagatgcaaacaccggccacacaggatctgagaagcatttccaggtctatgaataacaccacgaggagacaaaagcaaacacagcaaatgttctcaaataaagcaaggacattatagtccaaatttaatttttacctctaacaaaacttatgtattacatggttaagagaccaaggctacagttttcacatgtaaaaactgtagccattaagcaggttaaacttgttttagatcataccagaacagttgaaaattaacagcaatatctaatttcttgttccatagaatgaatgctatgagaaatatatcactggacgaggcttcctggagccaccccaagcctgtacatggcaagatggcagtgctgcaagcccactgcctgtacattcagtgtaagagcattcgtttttccattgagaacccctggctattaaaacaaactatcataattttatgttaaatcatagctgccaatcagaagaagtactctttctgattttcattgactgcattttgtatattaagctcacttttcagaacagcctcagcactgtctacattctctgacctttttgcctcacttcttttatataaccttttctgctgataaatgcgaacagctatggcagtgatgcaaagcaagataaaaatcacaacagctatcagacctccaattactgcagagtcacttttgattgcattagcaaggggctctctgtcatctattgttccagaatgatctgcaaacgagtgtgtcctttcccttgatgtggcatcagtgccaggctgggccatacagctggactcagtcacgtgtcctgtaacagtgacagggtctgggtggctggggtgcagagctgccttcagaggggccacgtggctgagctgcactgcagagaggcagcctgtgaagccctgcgcacctgccagtgcagtatcctggtccacatcactgtgttctaaaatcctgcccaataccagagatttgactgcactgaattctgtgcctgatgacaggtgaacttgtctccttctattatcgtcaatctctataaagaccactccttcttctctgttaatcattatgtggtgaagttgtccatcagccatgtttttaaaatcaaagttaacaacatcaggctcttgatatttatttaacttgtacctgatctgcaaacttccatttttggcaatgatcacagaaaggtattctttgtaaaaggagctcacaaaaagcagcaagcttggtgttcgtgttgttcggaaactaaatttgatcatttctctgctcagcttcatatcaccatgaaatgaagcagcgtgggagctggagtttttacttaaaagataattttcttgaaaattgtatatcacggatgagccagatccaaaatatgcagaaatctcatttgagcagaatggccctgtgtatgcagagaaagtgcagtcacaaaagaacccaatgggtctttctctgcatttccctccattgcggcataacttcccatagctgctgcaatgtcccctacaacctggctgcacttctggagtcacctgggctctttcttccaaatccagggtcatcccattcaactgcagagaccgaatgcagcccagaaagcctctctgtctggtggccgttccacccacgaagagctgactgttgagctgtaacaggacatgcccatcagcgggggcgggctgtgtctttggtgtcagctgatccacttgaagggaggcctccttcatgttcctttcaaccctcacatggtgccactggttgtcgttgaagtgggtgggtgactgcactgagatttcaaaaggcccattccccacatcaaatgaaaaagtcactactgtcggagagcgaagctctatccgtataaaatcagcaatccccaagttctctaaaaataccccagatgaagctgttgtcttaaaaaagaaagatacatccgcgctaagttctccgtggaaggtaggaaaatgaagatatgaagcctcggtatcaaaggaagctgaattccaaaatgatctgtctccctggcagagcagaggccccagtttataagctgcttctgaatgcagtcggcctgtgtctgtaatcacgatcttagttactggaagatgttctttataagcaagcaatccagtgtcattggtccattcattccggtcagcatcacaattgcagtaatactgagaatcaatgcagtttccctctaatccacaagtacatttttgaagatcaggcgaagaacctccccagtaggtttgcgtttcattggttcttcctacccaccaactcagaggggttccatcttgcttattgaccagccgtgacttcttgcagtaataagtaaactcctgttcacagtgctctgcacggttaatagtggcctgaagttgctccatgctggccacatactcgaaaaacccagcatatgggttctctggattagtatttctgactcttgttaagtcagagccgttgtgctgtatgatggtccatgcagtttcggtcatattgcaatatagaagaaatggttccaggggaccacttccatctgaatctatatagtaaaaccctgaagtatttcctctgtgcttataggcttcacatgactgctcatagatagagttatggcaagtagctcctctgtaaccagtgttggtacagttacaatgaaaggtgctccaggactgggaacactccccaccgtgttcacaatagttgggcaaacacctgtctgagatgccacatgagtctatctgaaggtcactgaagttcccaagggacccctgctgaactgaaatcagatctaccactttgccgctgatagaaatgagcctcatacatccctgaaatccaccaagtggacttttacatttggatccaaagcttttgtcaggacaacctgctgtgatgtcactgggtaattttcctggctggtagagattcgacttaagttttccatcactcagaaagaggaggataccccctgaaatcagctgaagttcactgaacagcagaagccctgccttattccaagttcgaaattgaaaagtggcagaaacctcctcctctccagagaagtctggcagtgctaaataactcctggagctcagaaaagtcacgggcatagattgtggttgtgaacaagaaaatgacacatttcccatagcaatgatctgtggtttttgctgcttggccaaatcaatgatatccactccattataatagagattttctaaacatccatgaaaatttctatgtgggaatgacactgattttccaggtgctggaatccctccaaagctgatctcataatcaagattcatgagattgaattctccccgtgcatggaaatgatgcctgtgttcgtccactgtgaagttgacttgtttgcccaaacgctggatgagcactgaatgccaatgctgatcatctagcaggctgcccagggtgagattgaccagggtggaagtggaaggcagtttagcttcacctgaattaataagtaaaaagagtcttgctcttcttaattgcagtgtgatgtgatctccatttggcccttccctgtggagtagaatcccatcactctgcatggttttgaatttcaaagaaataatgtcttttattgggctcagggatttttgatcaaatctgtagagaagggaactttttccatcaagatcaaccacttctgatctgtatgcacatccgaacacttcgattcgcattccaattctgcccttggggttccattccaaagggatgaagcgcagaaatctggctttgatagaaggctggagtctatagtacacaacactgtctgcatttgcatttcctgaaaaaccccagatgctgtcctcttggcgatattgtttccagttccagccactatcactgaacatcaggaggtagctggtcacccagttggagctaccatatcccccttgagtggccacagcggtgacctccattctctctccaaggtcaatctgcaaccactggtatttgttagacacaagtggagaccagccaccagctccatctcttctattcagccttgcaaatccaggaccatgactgctggagagctcggaagaactgctgaaggatgcctgaggcaaggcagacacaagaggatcatcacagtcataggaattcccagcttcgactctgttccaattttgagtagataacagaagtagcgtcttgaggacagctcccgtgacagatcccatgttcacatttattgggctcccccaaaagatcttgagaggctctcagagcgctccagtcctcttctcagtagctctgccagctctgtctgggtcttcagcccctctaggtctctgtctctccccctcccttcctcctcacctccctccgtcttttcttcttccctcctccctctcttctctctccctctctctctccccgtctctgtctctctcttttctctctctctctcacacacacctccctgactcctcactgaaaagc

SEQ ID NO: 19076 - RNA, 6369 nt, Homo sapiens
  source 1..6369: mol_type = other RNA
tgggagagaggactgtgaggcttcaccaataaacctccctagagttcagctaccaatgaggttaataccgctactaaataacatgaacatctgcaaaagattcagagatataatgatgtttgcactcagctttgcatcgaataaataatgccatttctatgttaaatccttcccttgtcaccatagatcttccaatcaaacaaagagtataccatctaccaacataggtccttagtccttcgtaaactactatgttaattcaggttcttaagatttagtcaggcatttgcagaaacatcaatatggatatagtgctatgagaaaagagaggcaggttttataagaagagttaacaaggaaaatatagaaaataagatgatagtaatgctaaatttacatatttcccgattcttctggtgtagacaaactaagaaatccaatagttacttgggaggcacttgaaggtgtgagtatgtataatagagtgcctttattgtatgattggcttgcagaattcaaagatagttccttgtatgcatggtctcaagattaattattgtaacagttccataaggttattgatcattctttgatctcctagtgtataatacaccctaatcagaatgtaccattcagcaagttggattgattcttggtaatttttgagaaattcaccccatcgtttcagacgagaagtgtctggaatgacaaattcacagtagatcatttaatatgctatctccccttagagtgtgcattgtttaattattgattgtgtagatcactgatggttgcagctcatatttcaaaaagtatgtactggaagtctatgcacagcaaaatgtacacctaaaggggtatatgtttcagaatgggaaatggggctctatacttcaatttgtctcttttttggtaatatataagatgattcgtgaagtataatcattgaagatcaaggcgaagtttgtgataaacttcagaaaaacagaaatgtaaaccaataaaggactgatctaggtttgggcaaaatagtctcataagtatatttcatttgaggtattacagttgtaaattaaataataattttttgctgtgttaagaattttttttaatatatcaacagtttagttgaaaacattttacattctttgggaaactggcattactcagggtcttaagtactgtcaccatcaaacaatggtagcaaattaattggaaaactttttttaaaaggaaagacattacatactaacaaccactgcactttctgagtcttgttaaatacaacttgtatgttcagagttgaagtctgagactcaaaaccaaatgtattcaacattattaagaagagacaaatagaataatgagcaatacaaacaaagcaaagacagcaaaacatttttcaagactattgatgtattgtattgaatataatacagagaaaggcaaaggggctttattatgcttgtggccactgaagatgcaaacaccggccacacaggatctgagaagcatttccaggtctatgaataacaccacgaggagacaaaagcaaacacagcaaatgttctcaaataaagcaaggacattatagtccaaatttaatttttacctctaacaaaacttatgtattacatggttaagagaccaaggctacagttttcacatgtaaaaactgtagccattaagcaggttaaacttgttttagatcataccagaacagttgaaaattaacagcaatatctaatttcttgttccatagaatgaatgctatgagaaatatatcactggacgaggcttcctggagccaccccaagcctgtacatggcaagatggcagtgctgcaagcccactgcctgtacattcagtgtaagagcattcgtttttccattgagaacccctggctattaaaacaaactatcataattttatgttaaatcatagctgccaatcagaagaagtactctttctgattttcattgactgcattttgtatattaagctcacttttcagaacagcctcagcactgtctacattctctgacctttttgcctcacttcttttatataaccttttctgctgataaatgcgaacagctatggcagtgatgcaaagcaagataaaaatcacaacagctatcagacctccaattactgcagagtcacttttgattgcattagcaaggggctctctgtcatctattgttccagaatgatctgcaaacgagtgtgtcctttcccttgatgtggcatcagtgccaggctgggccatacagctggactcagtcacgtgtcctgtaacagtgacagggtctgggtggctggggtgcagagctgccttcagaggggccacgtggctgagctgcactgcagagaggcagcctgtgaagccctgcgcacctgccagtgcagtatcctggtccacatcactgtgttctaaaatcctgcccaataccagagatttgactgcactgaattctgtgcctgatgacaggtgaacttgtctccttctattatcgtcaatctctataaagaccactccttcttctctgttaatcattatgtggtgaagttgtccatcagccatgtttttaaaatcaaagttaacaacatcaggctcttgatatttatttaacttgtacctgatctgcaaacttccatttttggcaatgatcacagaaaggtattctttgtaaaaggagctcacaaaaagcagcaagcttggtgttcgtgttgttcggaaactaaatttgatcatttctctgctcagcttcatatcaccatgaaatgaagcagcgtgggagctggagtttttacttaaaagataattttcttgaaaattgtatatcacggatgagccagatccaaaatatgcagaaatctcatttgagcagaatggccctgtgtatgcagagaaagtgcagtcacaaaagaacccaatgggtctttctctgcatttccctccattgcggcataacttcccatagctgctgcaatgtcccctacaacctggctgcacttctggagtcacctgggctctttcttccaaatccagggtcatcccattcaactgcagagaccgaatgcagcccagaaagcctctctgtctggtggccgttccacccacgaagagctgactgttgagctgtaacaggacatgcccatcagcgggggcgggctgtgtctttggtgtcagctgatccacttgaagggaggcctccttcatgttcctttcaaccctcacatggtgccactggttgtcgttgaagtgggtgggtgactgcactgagatttcaaaaggcccattccccacatcaaatgaaaaagtcactactgtcggagagcgaagctctatccgtataaaatcagcaatccccaagttctctaaaaataccccagatgaagctgttgtcttaaaaaagaaagatacatccgcgctaagttctccgtggaaggtaggaaaatgaagatatgaagcctcggtatcaaaggaagctgaattccaaaatgatctgtctccctggcagagcagaggccccagtttataagctgcttctgaatgcagtcggcctgtgtctgtaatcacgatcttagttactggaagatgttctttataagcaagcaatccagtgtcattggtccattcattccggtcagcatcacaattgcagtaatactgagaatcaatgcagtttccctctaatccacaagtacatttttgaagatcaggcgaagaacctccccagtaggtttgcgtttcattggttcttcctacccaccaactcagaggggttccatcttgcttattgaccagccgtgacttcttgcagtaataagtaaactcctgttcacagtgctctgcacggttaatagtggcctgaagttgctccatgctggccacatactcgaaaaacccagcatatgggttctctggattagtatttctgactcttgttaagtcagagccgttgtgctgtatgatggtccatgcagtttcttgtatgcagaaatggggggagaaagagaggagaccatcactagtcggtcatattgcaatatagaagaaatggttccaggggaccacttccatctgaatctatatagtaaaaccctgaagtatttcctctgtgcttataggcttcacatgactgctcatagatagagttatggcaagtagctcctctgtaaccagtgttggtacagttacaatgaaaggtgctccaggactgggaacactccccaccgtgttcacaatagttgggcaaacacctgtctgagatgccacatgagtctatctgaaggtcactgaagttcccaagggacccctgctgaactgaaatcagatctaccactttgccgctgatagaaatgagcctcatacatccctgaaatccaccaagtggacttttacatttggatccaaagcttttgtcaggacaacctccaaaataataggtgccacccgaataaatctgctcaggccccagcagaggagcagcagaagccatctggccgtccaccgccacactcaagtgattctttttagcagataaagagacagaatgccactgcccatcatttaattcgacacctgcccctggcatttctccgacatctcattctcaaagccctgtgtgcaagactctacttctcttatttcattttagactttccactggtgtccaacagttcttctcaaactatcttaaatacggagaaaatgaggctcagagaggaaaagaaactaccgaggtcacatccagctgctggatagctgctgtgatgtcactgggtaattttcctggctggtagagattcgacttaagttttccatcactcagaaagaggaggataccccctgaaatcagctgaagttcactgaacagcagaagccctgccttattccaagttcgaaattgaaaagtggcagaaacctcctcctctccagagaagtctggcagtgctaaataactcctggagctcagaaaagtcacgggcatagattgtggttgtgaacaagaaaatgacacatttcccatagcaatgatctgtggtttttgctgcttggccaaatcaatgatatccactccattataatagagattttctaaacatccatgaaaatttctatgtgggaatgacactgattttccaggtgctggaatccctccaaagctgatctcataatcaagattcatgagattgaattctccccgtgcatggaaatgatgcctgtgttcgtccactgtgaagttgacttgtttgcccaaacgctggatgagcactgaatgccaatgctgatcatctagcaggctgcccagggtgagattgaccagggtggaagtggaaggcagtttagcttcacctgaattaataagtaaaaagagtcttgctcttcttaattgcagtgtgatgtgatctccatttggcccttccctgtggagtagaatcccatcactctgcatggttttgaatttcaaagaaataatgtcttttattgggctcagggatttttgatcaaatctgtagagaagggaactttttccatcaagatcaaccacttctgatctgtatgcacatccgaacacttcgattcgcattccaattctgcccttggggttccattccaaagggatgaagcgcagaaatctggctttgatagaaggctggagtctatagtacacaacactgtctgcatttgcatttcctgaaaaaccccagatgctgtcctcttggcgatattgtttccagttccagccactatcactgaacatcaggaggtagctggtcacccagttggagctaccatatcccccttgagtggccacagcggtgacctccattctctctccaaggtcaatctgcaaccactggtatttgttagacacaagtggagaccagccaccagctccatctcttctattcagccttgcaaatccaggaccatgactgctggagagctcggaagaactgctgaaggatgcctgaggcaaggcagacacaagaggatcatcacagtcataggaattcccagcttcgactctgttccaattttgagtagataacagaagtagcgtcttgaggacagctcccgtgacagatcccatgttcacatttattgggctcccccaaaagatcttgagaggctctcagagcgctccagtcctcttctcagtagctctgccagctctgtctgggtcttcagcccctctaggtctctgtctctccccctcccttcctcctcacctccctccgtcttttcttcttccctcctccctctcttctctctccctctctctctccccgtctctgtctctctcttttctctctctctctcacacacacctccctgactcctcactgaaaagc

SEQ ID NO: 19077 - RNA, 6181 nt, Homo sapiens
  source 1..6181: mol_type = other RNA
tgggagagaggactgtgaggcttcaccaataaacctccctagagttcagctaccaatgaggttaataccgctactaaataacatgaacatctgcaaaagattcagagatataatgatgtttgcactcagctttgcatcgaataaataatgccatttctatgttaaatccttcccttgtcaccatagatcttccaatcaaacaaagagtataccatctaccaacataggtccttagtccttcgtaaactactatgttaattcaggttcttaagatttagtcaggcatttgcagaaacatcaatatggatatagtgctatgagaaaagagaggcaggttttataagaagagttaacaaggaaaatatagaaaataagatgatagtaatgctaaatttacatatttcccgattcttctggtgtagacaaactaagaaatccaatagttacttgggaggcacttgaaggtgtgagtatgtataatagagtgcctttattgtatgattggcttgcagaattcaaagatagttccttgtatgcatggtctcaagattaattattgtaacagttccataaggttattgatcattctttgatctcctagtgtataatacaccctaatcagaatgtaccattcagcaagttggattgattcttggtaatttttgagaaattcaccccatcgtttcagacgagaagtgtctggaatgacaaattcacagtagatcatttaatatgctatctccccttagagtgtgcattgtttaattattgattgtgtagatcactgatggttgcagctcatatttcaaaaagtatgtactggaagtctatgcacagcaaaatgtacacctaaaggggtatatgtttcagaatgggaaatggggctctatacttcaatttgtctcttttttggtaatatataagatgattcgtgaagtataatcattgaagatcaaggcgaagtttgtgataaacttcagaaaaacagaaatgtaaaccaataaaggactgatctaggtttgggcaaaatagtctcataagtatatttcatttgaggtattacagttgtaaattaaataataattttttgctgtgttaagaattttttttaatatatcaacagtttagttgaaaacattttacattctttgggaaactggcattactcagggtcttaagtactgtcaccatcaaacaatggtagcaaattaattggaaaactttttttaaaaggaaagacattacatactaacaaccactgcactttctgagtcttgttaaatacaacttgtatgttcagagttgaagtctgagactcaaaaccaaatgtattcaacattattaagaagagacaaatagaataatgagcaatacaaacaaagcaaagacagcaaaacatttttcaagactattgatgtattgtattgaatataatacagagaaaggcaaaggggctttattatgcttgtggccactgaagatgcaaacaccggccacacaggatctgagaagcatttccaggtctatgaataacaccacgaggagacaaaagcaaacacagcaaatgttctcaaataaagcaaggacattatagtccaaatttaatttttacctctaacaaaacttatgtattacatggttaagagaccaaggctacagttttcacatgtaaaaactgtagccattaagcaggttaaacttgttttagatcataccagaacagttgaaaattaacagcaatatctaatttcttgttccatagaatgaatgctatgagaaatatatcactggacgaggcttcctggagccaccccaagcctgtacatggcaagatggcagtgctgcaagcccactgcctgtacattcagtgtaagagcattcgtttttccattgagaacccctggctattaaaacaaactatcataattttatgttaaatcatagctgccaatcagaagaagtactctttctgattttcattgactgcattttgtatattaagctcacttttcagaacagcctcagcactgtctacattctctgacctttttgcctcacttcttttatataaccttttctgctgataaatgcgaacagctatggcagtgatgcaaagcaagataaaaatcacaacagctatcagacctccaattactgcagagtcacttttgattgcattagcaaggggctctctgtcatctattgttccagaatgatctgcaaacgagtgtgtcctttcccttgatgtggcatcagtgccaggctgggccatacagctggactcagtcacgtgtcctgtaacagtgacagggtctgggtggctggggtgcagagctgccttcagaggggccacgtggctgagctgcactgcagagaggcagcctgtgaagccctgcgcacctgccagtgcagtatcctggtccacatcactgtgttctaaaatcctgcccaataccagagatttgactgcactgaattctgtgcctgatgacaggtgaacttgtctccttctattatcgtcaatctctataaagaccactccttcttctctgttaatcattatgtggtgaagttgtccatcagccatgtttttaaaatcaaagttaacaacatcaggctcttgatatttatttaacttgtacctgatctgcaaacttccatttttggcaatgatcacagaaaggtattctttgtaaaaggagctcacaaaaagcagcaagcttggtgttcgtgttgttcggaaactaaatttgatcatttctctgctcagcttcatatcaccatgaaatgaagcagcgtgggagctggagtttttacttaaaagataattttcttgaaaattgtatatcacggatgagccagatccaaaatatgcagaaatctcatttgagcagaatggccctgtgtatgcagagaaagtgcagtcacaaaagaacccaatgggtctttctctgcatttccctccattgcggcataacttcccatagctgctgcaatgtcccctacaacctggctgcacttctggagtcacctgggctctttcttccaaatccagggtcatcccattcaactgcagagaccgaatgcagcccagaaagcctctctgtctggtggccgttccacccacgaagagctgactgttgagctgtaacaggacatgcccatcagcgggggcgggctgtgtctttggtgtcagctgatccacttgaagggaggcctccttcatgttcctttcaaccctcacatggtgccactggttgtcgttgaagtgggtgggtgactgcactgagatttcaaaaggcccattccccacatcaaatgaaaaagtcactactgtcggagagcgaagctctatccgtataaaatcagcaatccccaagttctctaaaaataccccagatgaagctgttgtcttaaaaaagaaagatacatccgcgctaagttctccgtggaaggtaggaaaatgaagatatgaagcctcggtatcaaaggaagctgaattccaaaatgatctgtctccctggcagagcagaggccccagtttataagctgcttctgaatgcagtcggcctgtgtctgtaatcacgatcttagttactggaagatgttctttataagcaagcaatccagtgtcattggtccattcattccggtcagcatcacaattgcagtaatactgagaatcaatgcagtttccctctaatccacaagtacatttttgaagatcaggcgaagaacctccccagtaggtttgcgtttcattggttcttcctacccaccaactcagaggggttccatcttgcttattgaccagccgtgacttcttgcagtaataagtaaactcctgttcacagtgctctgcacggttaatagtggcctgaagttgctccatgctggccacatactcgaaaaacccagcatatgggttctctggattagtatttctgactcttgttaagtcagagccgttgtgctgtatgatggtccatgcagtttcttgtatgcagaaatggggggagaaagagaggagaccatcactagtcggtcatattgcaatatagaagaaatggttccaggggaccacttccatctgaatctatatagtaaaaccctgaagtatttcctctgtgcttataggcttcacatgactgctcatagatagagttatggcaagtagctcctctgtaaccagtgttggtacagttacaatgaaaggtgctccaggactgggaacactccccaccgtgttcacaatagttgggcaaacacctgtctgagatgccacatgagtctatctgaaggtcactgaagttcccaagggacccctgctgaactgaaatcagatctaccactttgccgctgatagaaatgagcctcatacatccctgaaatccaccaagtggacttttacatttggatccaaagcttttgtcaggacaacctccaaaataataggtgccacccgaataaatctgctcaggccccagcagaggagcagcagaagccatctggccgtccaccgccacactcaagtgattctttttagcagataaagagacagaatgccactgcccatcatttaattcgacacctgctgtgatgtcactgggtaattttcctggctggtagagattcgacttaagttttccatcactcagaaagaggaggataccccctgaaatcagctgaagttcactgaacagcagaagccctgccttattccaagttcgaaattgaaaagtggcagaaacctcctcctctccagagaagtctggcagtgctaaataactcctggagctcagaaaagtcacgggcatagattgtggttgtgaacaagaaaatgacacatttcccatagcaatgatctgtggtttttgctgcttggccaaatcaatgatatccactccattataatagagattttctaaacatccatgaaaatttctatgtgggaatgacactgattttccaggtgctggaatccctccaaagctcataatcaagattcatgagattgaattctccccgtgcatggaaatgatgcctgtgttcgtccactgtgaagttgacttgtttgcccaaacgctggatgagcactgaatgccaatgctgatcatctagcaggctgcccagggtgagattgaccagggtggaagtggaaggcagtttagcttcacctgaattaataagtaaaaagagtcttgctcttcttaattgcagtgtgatgtgatctccatttggcccttccctgtggagtagaatcccatcactctgcatggttttgaatttcaaagaaataatgtcttttattgggctcagggatttttgatcaaatctgtagagaagggaactttttccatcaagatcaaccacttctgatctgtatgcacatccgaacacttcgattcgcattccaattctgcccttggggttccattccaaagggatgaagcgcagaaatctggctttgatagaaggctggagtctatagtacacaacactgtctgcatttgcatttcctgaaaaaccccagatgctgtcctcttggcgatattgtttccagttccagccactatcactgaacatcaggaggtagctggtcacccagttggagctaccatatcccccttgagtggccacagcggtgacctccattctctctccaaggtcaatctgcaaccactggtatttgttagacacaagtggagaccagccaccagctccatctcttctattcagccttgcaaatccaggaccatgactgctggagagctcggaagaactgctgaaggatgcctgaggcaaggcagacacaagaggatcatcacagtcataggaattcccagcttcgactctgttccaattttgagtagataacagaagtagcgtcttgaggacagctcccgtgacagatcccatgttcacatttattgggctcccccaaaagatcttgagaggctctcagagcgctccagtcctcttctcagtagctctgccagctctgtctgggtcttcagcccctctaggtctctgtctctccccctcccttcctcctcacctccctccgtcttttcttcttccctcctccctctcttctctctccctctctctctccccgtctctgtctctctcttttctctctctctctcacacacacctccctgactcctcactgaaaagc

SEQ ID NO: 19078 - RNA, 5900 nt, Homo sapiens
  source 1..5900: mol_type = other RNA
tgggagagaggactgtgaggcttcaccaataaacctccctagagttcagctaccaatgaggttaataccgctactaaataacatgaacatctgcaaaagattcagagatataatgatgtttgcactcagctttgcatcgaataaataatgccatttctatgttaaatccttcccttgtcaccatagatcttccaatcaaacaaagagtataccatctaccaacataggtccttagtccttcgtaaactactatgttaattcaggttcttaagatttagtcaggcatttgcagaaacatcaatatggatatagtgctatgagaaaagagaggcaggttttataagaagagttaacaaggaaaatatagaaaataagatgatagtaatgctaaatttacatatttcccgattcttctggtgtagacaaactaagaaatccaatagttacttgggaggcacttgaaggtgtgagtatgtataatagagtgcctttattgtatgattggcttgcagaattcaaagatagttccttgtatgcatggtctcaagattaattattgtaacagttccataaggttattgatcattctttgatctcctagtgtataatacaccctaatcagaatgtaccattcagcaagttggattgattcttggtaatttttgagaaattcaccccatcgtttcagacgagaagtgtctggaatgacaaattcacagtagatcatttaatatgctatctccccttagagtgtgcattgtttaattattgattgtgtagatcactgatggttgcagctcatatttcaaaaagtatgtactggaagtctatgcacagcaaaatgtacacctaaaggggtatatgtttcagaatgggaaatggggctctatacttcaatttgtctcttttttggtaatatataagatgattcgtgaagtataatcattgaagatcaaggcgaagtttgtgataaacttcagaaaaacagaaatgtaaaccaataaaggactgatctaggtttgggcaaaatagtctcataagtatatttcatttgaggtattacagttgtaaattaaataataattttttgctgtgttaagaattttttttaatatatcaacagtttagttgaaaacattttacattctttgggaaactggcattactcagggtcttaagtactgtcaccatcaaacaatggtagcaaattaattggaaaactttttttaaaaggaaagacattacatactaacaaccactgcactttctgagtcttgttaaatacaacttgtatgttcagagttgaagtctgagactcaaaaccaaatgtattcaacattattaagaagagacaaatagaataatgagcaatacaaacaaagcaaagacagcaaaacatttttcaagactattgatgtattgtattgaatataatacagagaaaggcaaaggggctttattatgcttgtggccactgaagatgcaaacaccggccacacaggatctgagaagcatttccaggtctatgaataacaccacgaggagacaaaagcaaacacagcaaatgttctcaaataaagcaaggacattatagtccaaatttaatttttacctctaacaaaacttatgtattacatggttaagagaccaaggctacagttttcacatgtaaaaactgtagccattaagcaggttaaacttgttttagatcataccagaacagttgaaaattaacagcaatatctaatttcttgttccatagaatgaatgctatgagaaatatatcactggacgaggcttcctggagccaccccaagcctgtacatggcaagatggcagtgctgcaagcccactgcctgtacattcagtgtaagagcattcgtttttccattgagaacccctggctattaaaacaaactatcataattttatgttaaatcatagctgccaatcagaagaagtactctttctgattttcattgactgcattttgtatattaagctcacttttcagaacagcctcagcactgtctacattctctgacctttttgcctcacttcttttatataaccttttctgctgataaatgcgaacagctatggcagtgatgcaaagcaagataaaaatcacaacagctatcagacctccaattactgcagagtcacttttgattgcattagcaaggggctctctgtcatctattgttccagaatgatctgcaaacgagtgtgtcctttcccttgatgtggcatcagtgccaggctgggccatacagctggactcagtcacgtgtcctgtaacagtgacagggtctgggtggctggggtgcagagctgccttcagaggggccacgtggctgagctgcactgcagagaggcagcctgtgaagccctgcgcacctgccagtgcagtatcctggtccacatcactgtgttctaaaatcctgcccaataccagagatttgactgcactgaattctgtgcctgatgacaggtgaacttgtctccttctattatcgtcaatctctataaagaccactccttcttctctgttaatcattatgtggtgaagttgtccatcagccatgtttttaaaatcaaagttaacaacatcaggctcttgatatttatttaacttgtacctgatctgcaaacttccatttttggcaatgatcacagaaaggtattctttgtaaaaggagctcacaaaaagcagcaagcttggtgttcgtgttgttcggaaactaaatttgatcatttctctgctcagcttcatatcaccatgaaatgaagcagcgtgggagctggagtttttacttaaaagataattttcttgaaaattgtatatcacggatgagccagatccaaaatatgcagaaatctccacgaagagctgactgttgagctgtaacaggacatgcccatcagcgggggcgggctgtgtctttggtgtcagctgatccacttgaagggaggcctccttcatgttcctttcaaccctcacatggtgccactggttgtcgttgaagtgggtgggtgactgcactgagatttcaaaaggcccattccccacatcaaatgaaaaagtcactactgtcggagagcgaagctctatccgtataaaatcagcaatccccaagttctctaaaaataccccagatgaagctgttgtcttaaaaaagaaagatacatccgcgctaagttctccgtggaaggtaggaaaatgaagatatgaagcctcggtatcaaaggaagctgaattccaaaatgatctgtctccctggcagagcagaggccccagtttataagctgcttctgaatgcagtcggcctgtgtctgtaatcacgatcttagttactggaagatgttctttataagcaagcaatccagtgtcattggtccattcattccggtcagcatcacaattgcagtaatactgagaatcaatgcagtttccctctaatccacaagtacatttttgaagatcaggcgaagaacctccccagtaggtttgcgtttcattggttcttcctacccaccaactcagaggggttccatcttgcttattgaccagccgtgacttcttgcagtaataagtaaactcctgttcacagtgctctgcacggttaatagtggcctgaagttgctccatgctggccacatactcgaaaaacccagcatatgggttctctggattagtatttctgactcttgttaagtcagagccgttgtgctgtatgatggtccatgcagtttcggtcatattgcaatatagaagaaatggttccaggggaccacttccatctgaatctatatagtaaaaccctgaagtatttcctctgtgcttataggcttcacatgactgctcatagatagagttatggcaagtagctcctctgtaaccagtgttggtacagttacaatgaaaggtgctccaggactgggaacactccccaccgtgttcacaatagttgggcaaacacctgtctgagatgccacatgagtctatctgaaggtcactgaagttcccaagggacccctgctgaactgaaatcagatctaccactttgccgctgatagaaatgagcctcatacatccctgaaatccaccaagtggacttttacatttggatccaaagcttttgtcaggacaacctccaaaataataggtgccacccgaataaatctgctcaggccccagcagaggagcagcagaagccatctggccgtccaccgccacactcaagtgattctttttagcagataaagagacagaatgccactgcccatcatttaattcgacacctgctgtgatgtcactgggtaattttcctggctggtagagattcgacttaagttttccatcactcagaaagaggaggataccccctgaaatcagctgaagttcactgaacagcagaagccctgccttattccaagttcgaaattgaaaagtggcagaaacctcctcctctccagagaagtctggcagtgctaaataactcctggagctcagaaaagtcacgggcatagattgtggttgtgaacaagaaaatgacacatttcccatagcaatgatctgtggtttttgctgcttggccaaatcaatgatatccactccattataatagagattttctaaacatccatgaaaatttctatgtgggaatgacactgattttccaggtgctggaatccctccaaagctgatctcataatcaagattcatgagattgaattctccccgtgcatggaaatgatgcctgtgttcgtccactgtgaagttgacttgtttgcccaaacgctggatgagcactgaatgccaatgctgatcatctagcaggctgcccagggtgagattgaccagggtggaagtggaaggcagtttagcttcacctgaattaataagtaaaaagagtcttgctcttcttaattgcagtgtgatgtgatctccatttggcccttccctgtggagtagaatcccatcactctgcatggttttgaatttcaaagaaataatgtcttttattgggctcagggatttttgatcaaatctgtagagaagggaactttttccatcaagatcaaccacttctgatctgtatgcacatccgaacacttcgattcgcattccaattctgcccttggggttccattccaaagggatgaagcgcagaaatctggctttgatagaaggctggagtctatagtacacaacactgtctgcatttgcatttcctgaaaaaccccagatgctgtcctcttggcgatattgtttccagttccagccactatcactgaacatcaggaggtagctggtcacccagttggagctaccatatcccccttgagtggccacagcggtgacctccattctctctccaaggtcaatctgcaaccactggtatttgttagacacaagtggagaccagccaccagctccatctcttctattcagccttgcaaatccaggaccatgactgctggagagctcggaagaactgctgaaggatgcctgaggcaaggcagacacaagaggatcatcacagtcataggaattcccagcttcgactctgttccaattttgagtagataacagaagtagcgtcttgaggacagctcccgtgacagatcccatgttcacatttattgggctcccccaaaagatcttgagaggctctcagagcgctccagtcctcttctcagtagctctgccagctctgtctgggtcttcagcccctctaggtctctgtctctccccctcccttcctcctcacctccctccgtcttttcttcttccctcctccctctcttctctctccctctctctctccccgtctctgtctctctcttttctctctctctctcacacacacctccctgactcctcactgaaaagc

SEQ ID NO: 19079 - RNA, 6282 nt, Homo sapiens
  source 1..6282: mol_type = other RNA
tgggagagaggactgtgaggcttcaccaataaacctccctagagttcagctaccaatgaggttaataccgctactaaataacatgaacatctgcaaaagattcagagatataatgatgtttgcactcagctttgcatcgaataaataatgccatttctatgttaaatccttcccttgtcaccatagatcttccaatcaaacaaagagtataccatctaccaacataggtccttagtccttcgtaaactactatgttaattcaggttcttaagatttagtcaggcatttgcagaaacatcaatatggatatagtgctatgagaaaagagaggcaggttttataagaagagttaacaaggaaaatatagaaaataagatgatagtaatgctaaatttacatatttcccgattcttctggtgtagacaaactaagaaatccaatagttacttgggaggcacttgaaggtgtgagtatgtataatagagtgcctttattgtatgattggcttgcagaattcaaagatagttccttgtatgcatggtctcaagattaattattgtaacagttccataaggttattgatcattctttgatctcctagtgtataatacaccctaatcagaatgtaccattcagcaagttggattgattcttggtaatttttgagaaattcaccccatcgtttcagacgagaagtgtctggaatgacaaattcacagtagatcatttaatatgctatctccccttagagtgtgcattgtttaattattgattgtgtagatcactgatggttgcagctcatatttcaaaaagtatgtactggaagtctatgcacagcaaaatgtacacctaaaggggtatatgtttcagaatgggaaatggggctctatacttcaatttgtctcttttttggtaatatataagatgattcgtgaagtataatcattgaagatcaaggcgaagtttgtgataaacttcagaaaaacagaaatgtaaaccaataaaggactgatctaggtttgggcaaaatagtctcataagtatatttcatttgaggtattacagttgtaaattaaataataattttttgctgtgttaagaattttttttaatatatcaacagtttagttgaaaacattttacattctttgggaaactggcattactcagggtcttaagtactgtcaccatcaaacaatggtagcaaattaattggaaaactttttttaaaaggaaagacattacatactaacaaccactgcactttctgagtcttgttaaatacaacttgtatgttcagagttgaagtctgagactcaaaaccaaatgtattcaacattattaagaagagacaaatagaataatgagcaatacaaacaaagcaaagacagcaaaacatttttcaagactattgatgtattgtattgaatataatacagagaaaggcaaaggggctttattatgcttgtggccactgaagatgcaaacaccggccacacaggatctgagaagcatttccaggtctatgaataacaccacgaggagacaaaagcaaacacagcaaatgttctcaaataaagcaaggacattatagtccaaatttaatttttacctctaacaaaacttatgtattacatggttaagagaccaaggctacagttttcacatgtaaaaactgtagccattaagcaggttaaacttgttttagatcataccagaacagttgaaaattaacagcaatatctaatttcttgttccatagaatgaatgctatgagaaatatatcactggacgaggcttcctggagccaccccaagcctgtacatggcaagatggcagtgctgcaagcccactgcctgtacattcagtgtaagagcattcgtttttccattgagaacccctggctattaaaacaaactatcataattttatgttaaatcatagctgccaatcagaagaagtactctttctgattttcattgactgcattttgtatattaagctcacttttcagaacagcctcagcactgtctacattctctgacctttttgcctcacttcttttatataaccttttctgctgataaatgcgaacagctatggcagtgatgcaaagcaagataaaaatcacaacagctatcagacctttctttacactctgaatatgatatggatatagaaagtaaacaattatcctgttgccctgccagggagatacaattttaaagtttttgtgccagtaatacgattattcatatatgatatgaataaataacaagttgagcacctccaattactgcagagtcacttttgattgcattagcaaggggctctctgtcatctattgttccagaatgatctgcaaacgagtgtgtcctttcccttgatgtggcatcagtgccaggctgggccatacagctggactcagtcacgtgtcctgtaacagtgacagggtctgggtggctggggtgcagagctgccttcagaggggccacgtggctgagctgcactgcagagaggcagcctgtgaagccctgcgcacctgccagtgcagtatcctggtccacatcactgtgttctaaaatcctgcccaataccagagatttgactgcactgaattctgtgcctgatgacaggtgaacttgtctccttctattatcgtcaatctctataaagaccactccttcttctctgttaatcattatgtggtgaagttgtccatcagccatgtttttaaaatcaaagttaacaacatcaggctcttgatatttatttaacttgtacctgatctgcaaacttccatttttggcaatgatcacagaaaggtattctttgtaaaaggagctcacaaaaagcagcaagcttggtgttcgtgttgttcggaaactaaatttgatcatttctctgctcagcttcatatcaccatgaaatgaagcagcgtgggagctggagtttttacttaaaagataattttcttgaaaattgtatatcacggatgagccagatccaaaatatgcagaaatctcatttgagcagaatggccctgtgtatgcagagaaagtgcagtcacaaaagaacccaatgggtctttctctgcatttccctccattgcggcataacttcccatagctgctgcaatgtcccctacaacctggctgcacttctggagtcacctgggctctttcttccaaatccagggtcatcccattcaactgcagagaccgaatgcagcccagaaagcctctctgtctggtggccgttccacccacgaagagctgactgttgagctgtaacaggacatgcccatcagcgggggcgggctgtgtctttggtgtcagctgatccacttgaagggaggcctccttcatgttcctttcaaccctcacatggtgccactggttgtcgttgaagtgggtgggtgactgcactgagatttcaaaaggcccattccccacatcaaatgaaaaagtcactactgtcggagagcgaagctctatccgtataaaatcagcaatccccaagttctctaaaaataccccagatgaagctgttgtcttaaaaaagaaagatacatccgcgctaagttctccgtggaaggtaggaaaatgaagatatgaagcctcggtatcaaaggaagctgaattccaaaatgatctgtctccctggcagagcagaggccccagtttataagctgcttctgaatgcagtcggcctgtgtctgtaatcacgatcttagttactggaagatgttctttataagcaagcaatccagtgtcattggtccattcattccggtcagcatcacaattgcagtaatactgagaatcaatgcagtttccctctaatccacaagtacatttttgaagatcaggcgaagaacctccccagtaggtttgcgtttcattggttcttcctacccaccaactcagaggggttccatcttgcttattgaccagccgtgacttcttgcagtaataagtaaactcctgttcacagtgctctgcacggttaatagtggcctgaagttgctccatgctggccacatactcgaaaaacccagcatatgggttctctggattagtatttctgactcttgttaagtcagagccgttgtgctgtatgatggtccatgcagtttcggtcatattgcaatatagaagaaatggttccaggggaccacttccatctgaatctatatagtaaaaccctgaagtatttcctctgtgcttataggcttcacatgactgctcatagatagagttatggcaagtagctcctctgtaaccagtgttggtacagttacaatgaaaggtgctccaggactgggaacactccccaccgtgttcacaatagttgggcaaacacctgtctgagatgccacatgagtctatctgaaggtcactgaagttcccaagggacccctgctgaactgaaatcagatctaccactttgccgctgatagaaatgagcctcatacatccctgaaatccaccaagtggacttttacatttggatccaaagcttttgtcaggacaacctccaaaataataggtgccacccgaataaatctgctcaggccccagcagaggagcagcagaagccatctggccgtccaccgccacactcaagtgattctttttagcagataaagagacagaatgccactgcccatcatttaattcgacacctgctgtgatgtcactgggtaattttcctggctggtagagattcgacttaagttttccatcactcagaaagaggaggataccccctgaaatcagctgaagttcactgaacagcagaagccctgccttattccaagttcgaaattgaaaagtggcagaaacctcctcctctccagagaagtctggcagtgctaaataactcctggagctcagaaaagtcacgggcatagattgtggttgtgaacaagaaaatgacacatttcccatagcaatgatctgtggtttttgctgcttggccaaatcaatgatatccactccattataatagagattttctaaacatccatgaaaatttctatgtgggaatgacactgattttccaggtgctggaatccctccaaagctgatctcataatcaagattcatgagattgaattctccccgtgcatggaaatgatgcctgtgttcgtccactgtgaagttgacttgtttgcccaaacgctggatgagcactgaatgccaatgctgatcatctagcaggctgcccagggtgagattgaccagggtggaagtggaaggcagtttagcttcacctgaattaataagtaaaaagagtcttgctcttcttaattgcagtgtgatgtgatctccatttggcccttccctgtggagtagaatcccatcactctgcatggttttgaatttcaaagaaataatgtcttttattgggctcagggatttttgatcaaatctgtagagaagggaactttttccatcaagatcaaccacttctgatctgtatgcacatccgaacacttcgattcgcattccaattctgcccttggggttccattccaaagggatgaagcgcagaaatctggctttgatagaaggctggagtctatagtacacaacactgtctgcatttgcatttcctgaaaaaccccagatgctgtcctcttggcgatattgtttccagttccagccactatcactgaacatcaggaggtagctggtcacccagttggagctaccatatcccccttgagtggccacagcggtgacctccattctctctccaaggtcaatctgcaaccactggtatttgttagacacaagtggagaccagccaccagctccatctcttctattcagccttgcaaatccaggaccatgactgctggagagctcggaagaactgctgaaggatgcctgaggcaaggcagacacaagaggatcatcacagtcataggaattcccagcttcgactctgttccaattttgagtagataacagaagtagcgtcttgaggacagctcccgtgacagatcccatgttcacatttattgggctcccccaaaagatcttgagaggctctcagagcgctccagtcctcttctcagtagctctgccagctctgtctgggtcttcagcccctctaggtctctgtctctccccctcccttcctcctcacctccctccgtcttttcttcttccctcctccctctcttctctctccctctctctctccccgtctctgtctctctcttttctctctctctctcacacacacctccctgactcctcactgaaaagc

SEQ ID NO: 19080 - RNA, 65 nt, Homo sapiens
  source 1..65: mol_type = other RNA
tgggagctaagctatgggtatgcagatgcatacataagctcagtatacccatagcttagctccca

SEQ ID NO: 19081 - RNA, 1544 nt, Homo sapiens
  source 1..1544: mol_type = other RNA
tgggaggaggggatcttgggagtgatcccaacagctgagctccctgaatccctgtcccagcaggtgcatcccggccccacgccccaggcacccctgcaggccgagtccgcccggaactcaagaccaagcagcagatcctgaagcagcggcgccgggcccagaagctgcacttcctgcagcgtggtggcctcaagcagctctctgcccgcaaccgccgccgcgtccaggagctgcagcagggcgccttcggccggggtgcccgctccaagaagggcaagatgcggaagaggatgtgaggaccaggacccagccccgtggctccttgattggccttagggtgggcatcagcagacgttcccgtgcaccactgtgtgcctggccctgtgctgggcactgggggcactccctgcaggagccatcatctgtgaaaaggagcactgtatggccacagaagggcagcagctgcgtcagcctgtgtcagggctaggaggcaggggctgcaggctcagcctgacccaggccggccagcatggcagagaggtcctgcatgaacagcttcacgtgctctagctgtccctccgtgtcctcgatgtccagggtgggaggctgcccctgatgctggcacactagctggaacaggttgagcacagccatcctgctgcgtcccaggagcagagtcttctccgctgctgtgttctgaatctgaatccacttggattcccactgcagcgtacgctccctggcagcctccaggcgctcctgcagctgtgcccgccgctggccctgtgcgagcacctcgtccggccaggcgtcccgcagctgctgcagccgcgctcgcgccgcctccagctccgcgagctgctcgcgctccctgagcctcagcgccgcctgcgtctcggccaggccgtcgaagcgcgccaccagctccggaacctcttggaacccgggcagcagctccagcgcttgctccagcaggcgcgcgcagggctccaggcgcttaagccggcgctgcagccgcgcgtgttcccgccgtagctcctggagctgggtccacagacgcagcgcctccacctcccgacggcccgcctggtgcctctcctccgccgccctccgcagcgcgcgattgcgccgggcctcggagtcctgcaaaaacttgtcaaagcggatgaacgatccctttagctcccgctccttttgttccagctgttcccaacgctgtttcagggctgccgtcttggtgcggaacacctccttctgggcctgcagggcctggtctgcatctaccagctcttgcctcttctccaggagacgcagtactggtgggacatgatcctcagcctgctctggcagctttgtagacagtttctcttgcaaagccagtcggaaatattcctcccagggcaccgccatccttctggcagttgccccagctttctttccaccagctggagttttgcacaagcttaggagaccctgggggttctgtggagcgtggtgtggaagcctgctcagctcggcccagaaggcagccaccagcaggctct

SEQ ID NO: 19082 - RNA, 2739 nt, Homo sapiens
  source 1..2739: mol_type = other RNA
tgggaggggagaggcagcaagcagtcccgttcccacctgccctgctacttgtgggcctctgcatcctcgcccttgggtggggctgccaccgtggaggtggccttgaggctccgctttcgcttctgcacattctgctctggatggaagaggatgacgtaggttttgggtacgtagagcatgccgagggacaccgaggcactcaggctcaaggacacggttagcgtggttgtctggatgtagatcttttcagctgactgggcagtgccaaagaagatgggcacgaatgccagccagatgatgcaggtggtgtacatggtgaagccgatgggcttggcctcgttgaaggtctcgggcacgccacgggccttgatggcgtacactgtgcacgtgaccatgagcaggaggctgtagcccaggcagccgatgagagacagatccgacatgtcgcacttgagcacccctctggcctgctcggggtccaccgtccgctgttcctcatagtcaatcacgctgtgtgggggccgggcccccagccatgctatcatccccaccacctgcagggaggtgaggctgaaggtgatgaccagctgtgaggtggggctgatgaagggagggggtgtgaccgagcgcttgccctgctcaaagatgcggtagatacggttggtcttggtgagcagggcagagtagctgagggtcgtgcccaggcccaggaagagcctgcgggcggcacagaccgcggccccaggctcagccaccatgaggaaggtgatggcgtagatgaggaagatgccggtgaggaggacgtagctgagctctcggcccgaggcccggacgatgggcgtgttgttgtaccgcacgaaggtggccaccaccgtggtagtggccacgatgcccagcacggccaggaggagcggcggggctgcccagggggaggaccagctcaggcgcaccacaggtgtggggcggcagcccgtgtggttgggcgtgggcctcatgtccccaggacaggcctcgcatgtgaactcgtccacctggaagcggtacccgtcacaggcctcgcagtgccaacagcaggggacgcccttcaccatcttcttccgctcccccggcccgcagggcaggctgcacagagacgagggcacctcgtgggggtcgccagaccactgcagggcctccacatccagtctgagggtctctgcccactggcccactgcctggtacccgccactgctggcactgccattggtcgcctggtactggaagatgtcgtaccgcccgggcgcatctccgttctcgttgaacatcacaggggttcctgcgctgccattgaagcggacagctcgaatgtactgcagaagcatccgcccatcagtgggttccatcgccgggcacaggcctgtgtgcccagggcagagcgcctggtgcatgctgtggagggcgtgggcaatggcgtacaccgcatcaatcacaaactgcaccttgccctcctgctcgtaggtggagtcccggccgatgcgttcctcgcctgtgcatttgcgggtggaatcgtctgactgggtacctgagctggtcagtttgcagttaaaattctcttcccagaactcggcgaaccagatgttcctgcggttgttctccagggatcgagtcatgaagtactggtcaaatccgtcgatggaggcccttttgggcaggatggtgatggccccaacggccacgtcctccaggctcaagatgggtgaggtcttggctccccagctgtctgagccgacccacaggaagtggccggtcaggttggcctggcgagctgcctccaggacccgcctgatgtcatcctcattggcaaagatgatgatgccccgggcgttgggcgtctccatgagtctcctgatcaccttgctgaactctcctggctttggttccctgggaatcttgatagactgggcaatacagacccccccagcctctcgggagatctgaacgaaggcctcaaccccactttcgccatagttgccctcggaggccagcgtggacacatagttccatcccagtgccctcacgatgtccaccatggcctgcgcctggtaggagtcgggtggcaccacccgggagaagaagtcatagcgtgtggagtcgctgagctccggggctgtggaggcatagctgatctggggtatcgcaaacaggcgcagcacgttggcgaccatgatggagacggagctggccgaggcgcccacgacggccacgacgcgctcggggggcgcggggcgcagcggagggacgcctcccgggcagcgcacgcccacctcgtcgccgtcgccgcggccgcggatcagcgcctgcacgaagctcagcgcctgctccagcgcgtaggtgtcccgcgagcaggtgtccagcagccgcgcgcccaggcgcacgccgggcagcagctcggggtcggcgttgacgcggtccagcgcgtacagcatggcctccagccggtgcacgccctgctccttcttcagctgcccgcacgcccggcccgccgcgccccgcgcgtgcaccgggaacaggccgcccagcgtcaggccgcccgccaggcgcacagagcccgccgcgcgcgccaggcccgcctgcgccagccacgccagcggcagcagcgccacgagcagcggctcccgggctctccggggccgcgccatcggctcgtctagcgggctgcgccagccgctgtcggttcaggacaagtctgtgacagatgcg

SEQ ID NO: 19083 - RNA, 683 nt, Homo sapiens
  source 1..683: mol_type = other RNA
tgggccagggagcagctggtgggaggcgggagatgtgcaggctgagcacaggctcatgtgtgcgatgactcaggtccctcactggagacaccagctgagaggagagactgcagggcctggcacacacagggccactcttcctgctgccggccagaaggagctgatggaattaaccatcttcccgggagcaagactgagcccatggagggtgctgtggagcttgctgcaggttctgctggataggaaattgtgtctcatccacctgctgtctgcttctgtcctgtcttagcccagcagagctgttttaacacagacatttgcagcctgcccagtactctcctggatggatggtccccctcacggtggccttggaacccgcttcagcgggagaggcagcgcctcactcacggctccccctggccgctgctttaccagggagcgccaccccgtgccccgccagaggaagtgcaggcgccagcacagcacgggccgaaagccacactgtgggacccgcagcgcagctccaagaaatccaaagtccattcacaagaggagcttctccgccaaatcgttgaaaaataaaacgagaaatgagtcgccaccggtatccgctttagtcagccgtacgaaaacgcaacccggtcagctgcacttctgctgccagccctcctccagtcaagcac

SEQ ID NO: 19084 - RNA, 973 nt, Homo sapiens
  source 1..973: mol_type = other RNA
tgggccagggagcagctggtgggggcataggccaggtggatgttggccagtgtgatcctgtgtgtcaaggccatttcttgggacaccacgaggacgaagtagccatctctgaagcactggacagtagctgtgttgccatagtaacagggaacctctctggtgttgtcatagcagcagccagcctgctgacaggcttcttttgaagttcttctcacgatgcaggggaggtgccctgaggccacctggcactgctcctggctcaggtgggtacctatgtaatctcgtttgttcacatcccagtgttccaaggtgccccagtggggttgagccagggtggcgagggtaggtccaggtccaggggatggtaaagcaggggttgggtggacagagctgtgccctgggtccagtgggctgggaaaggcatggccagagccttgggaggtatggccagaggtggggaggaaggaaagggtttgtggggttgagacagagaacatggcgggtggtgccagctgggagtccagagtccgggaggggtcaggtttgggacagatcagagtagcgtcttgtgccacatccacacgaccattgggcagcacagcctccatgaacaccctcaggtggaaacgcccatccttctccagcacgtggcagcctctgtaatcggccgagaagactgcaggctcctgcggcctggaggtgacccagtggtagcagatggagcagttgttgacatcaaatcggttcccaaattcatccaccaccttgaagcggagagtctggcctggcctggggaacaccagcagctgcattcccttgatcccacagtcgtagctgtgccggaggcctgggaggccagggtcgggctggagccacctacccagccccagggtggcaaccagcagtagcagggccacagggtaaccccaggtcgtggctgagcctcctgccatgagacgccacagacacaccc

SEQ ID NO: 19085 - RNA, 352 nt, Homo sapiens
  source 1..352: mol_type = other RNA
tgggccagggagcagctggtgggggcataggccaggtggatgttggccagtgtgatcctgtgtgtcaaggccatttcttgggacaccacgaggacgaagtagccatctctgaagcactggacagtagctgtgttgccatagtaacagggaacctctctggtgttgtcatagcagcagccagcctgctgacaggcttcttttgaagttcttctcacgatgcaggggaggtgccctgaggccacctggcactgctcctggctcaggtgggtaccttctccagcacgtggcagcctctgtaatcggccgagaagactgcaggctcctgcggcctggaggtgacccagtggtagca

SEQ ID NO: 19086 - RNA, 489 nt, Homo sapiens
  source 1..489: mol_type = other RNA
tgggccagggagcagctggtgggggcataggccaggtggatgttggccagtgtgatcctgtgtgtcaaggccatttcttgggacaccacgaggacgaagtagccatctctgaagcactggacagtagtctccacttaggctggtgttggccccagcaaaccctttatggactgattttctcatccatgtgacaaatgagttgaactacactctaaaagtaggttcaccatataatctgtcatccaaaccagggcgtttcagatctgaaagtccagatgtgtgtaaggtagatctattaatagttccctgggacagttgttataaggccagctgggacatgtgaccgccccatctaaaggtctcctctgccatctgctctgggagttgggctctccaggaggaggataggaagcagtttccaccagctggaggagacagctctccttccgcttcagaatccaagggaccaggatcttgctggggtgggag

SEQ ID NO: 19087 - RNA, 1564 nt, Homo sapiens
  source 1..1564: mol_type = other RNA
tgggcgaggggtgggctctcagagatcgaggcgcgaatgcagcgcgccggtcttgctgtcgtggtcccagtaagagcaatgcatcatggcgagctcgggctgccgggcacaagcgaactgcaggcccggcgcactggtgggcgcgggcgccgggggcgcggcggtggctgggctggcagggctgagctggcccggcggcggcgcggcggccccgtggtgcggtggggcaggcggcggtgcggcggccgcgtgcagatggtgtgcgtgcggatgcgggtgggggtgcggcggaggcgggggtgcggccggcgggcctcccaggccattgtacgagttcactacgccggggggcagcgccatgctctgcacgcgtgtgtacggcccgtacgaggcggccgggcccgccagccccttgaccacagcggccgcgccagggctaccggggcccgcggctgcagccgcagctgctgcagccgctgcggctgccgccatctggcaggaggcatagggcatgggtgagggaggctgcggtagcggccacgagttgttgaggaagccagactgcaggtacttggggggcgccaggtagccgtagccgtcggccccggcgcccgccacgccgcacccgcctgcggcgcctccggccccgaagagccccttgccgggctggaagtgcgcgggcggcggccggaagggcctcttcatgcggcggcggcgccggtagttgcccttctcgaacatgtcttcgcaggccgggtccagcgtccagtagttgcccttgcgctcgccgccgccctcgcgcggcaccttgatgaagcactcgttgaggctgaggttgtggcggatgctattttgccagcccttcttattcttctcgtagaacgggaacttcgcgatgatgtactggtagatgccggacagcgtgagcctcttctccgcgctctcgcggatcgccatggcgatgagcgccacgtacgagtacgggggcttctgcgccgggtccggcttctccggggctgtcccgccgccacccccaccgcccttgcctgggctcggcggcggcccttctggctccttgactgtgcgaccggtctctggggccagcagggcccccgccgcgtcctcgggctcggggtagctggccatcatgacaaagccggcgcgccgcggccgggccgcctctgctctccgctccaggcgctggcgcggcaaagagttggggcgcacgagtccgcttacggccaagtctcaaacttctggagactgcggatgccgcccgcgcttgcttgctggaggcctgtcgctgctctcccctctccttccccttcccctagggagcggccggcgggagtggagctcagcctctggccatggggagtccgcccaacagagaggggctccggcctcgccgcccctccccgctcaggccagtccccgccttggtgggttttcttttctgcgctcttcccctccccccgccccccggtttcccgaagcacgacccgcgtctctggcggagctgcctcctggagtccctagtgcgccaggagcctcgctctgttct

SEQ ID NO: 19088 - RNA, 412 nt, Homo sapiens
  source 1..412: mol_type = other RNA
tgggcgcgccgggactgtgagacgacaggctgtggacgtgtccccacttcgccgtgtgaatcaggccatctggctgctgtgcacaggtgctcgtgaggctgccttccggaacattaagaccattgctgagtgcctggcagaggagctcatcaatgctgccaagggctcctccaactcctatgccattaagaagaaggacgtgtggccttcttggagcatgtggccaagtccaaccgctgattttcccagctgttgcccaataaacctgtctgcccttcagggcagccatgcttgagtctggtctacatccatttacgtaagtaaaactccccttccagactgacgaaattctttttgtgacaagaagacaaaggaatacgatggattgataagcgtagtcaaccgcgcagag

SEQ ID NO: 19089 - RNA, 500 nt, Homo sapiens
  source 1..500: mol_type = other RNA
tgggcgcgccgggactgtgagacgacaggctgtggacgtgtccccacttcgccgtgtgaatcaggccatctggctgctgtgcacaggtgctcgtgaggctgccttccggaacattaagaccattgctgagtgcctggcagaggagctcatcaatgctgccaagggctcctccaactcctatgccattaagaagaaggacgtgtggccttcttggagcatgtggccaagtccaaccgctgattttcccagctgttgcccaataaacctgtctgcccttcagggcagcccttaaagtaaatattttcagaaacaataggttaggtgccttagaaattcattcagaggcttagaaatccacattaacacagttcttacatgcttgagtctggtctacatccatttacgtaagtaaaactccccttccagactgacgaaattctttttgtgacaagaagacaaaggaatacgatggattgataagcgtagtcaaccgcgcagag

SEQ ID NO: 19090 - RNA, 2787 nt, Homo sapiens
  source 1..2787: mol_type = other RNA
tgggctgagggcaggaggcctgtggcggcggtgatgatggggagcaatgccacatcctggcagtggggtagaggagctggggacgtggccagggctggctccgaagtgtgaggggctcttctggtgcctctcggagctgcagtggattatcacgcatttggctgccattaccaaggggaaggccaggttgatctcagcaccgccctgaacaggtgatgcaggagatgccctcggcgctcaggttgtacttgaggtccagcagcacctggatgttggtatcaggccggaagagtagcggggcccggctggcggggcggagccggctggcgaacaccagggacaagatgaggatggagacgaacagccccacaatcacccagcggctcttgacggctgaccacaggacccagtggtgcagcagctcctgcagctgcacgatgagatggccgcggctgcccgtgttggaggctggctgcagaccctcgggggacacagacaccagggacacgtctcccagctccagtgacactggctcttcctcgacctccagcaaggggatgtcatcatccaggtagggtatggggccctgggcagggctgcctccaacctgctcgggagcggcaaacacgtctccggggaagtgcagggaggtcttccggctgcaattctggtggcagctggtctggcaggagctctccagtggtgccaggtagaggctccagaggcccagagctgcaggcatggtgacaagcacggccagccagcaacaggacacgatgagagacatgaacaggccaaagtcgtggacggctgggatctgggagaagacgttagctgcgtaggcggcggctgtggtcagggaggtgaagaaggtggccttgcctgcagtttggacggtgtggatcatgcgcagctgtgggtcttccaggtgggtggcctggcggtaggtgttgatgaacacaaagacatcgtccacaccaatgcccacgatcacgaaggcggccaccccattcaggatgcccaagtactggataccaaagaccacgtggtacaggaagagggccaccaggcagctgagaccaatgctggcaatcccaaagaaggacaggaacactgagcaggaggtgaggatgtagaccagggcagcaatgcagctgctgctgatgaaggccaggagcatgtcattgttgaacgtcctgcgcacttcatagtcaaacaggtctgtccccccatagagaacctggactttgctggtagactgcttggccagcatggccacgtaggtgaccacgaagctctgaaacttagcccgttgttcctcccagcggtcatctactgagtagtagttgggcaggggtgctccaaacaggatctcactgcgcaggagggagctcttcagattgtctgcagagaggccctcatccacataccagtagaactcagggtgagtcatggccagctccagggagccccggatgtccgccaggtcctggcccatgccgtcatagtagatcttgccgcccctctcggtgggaaaaaagtaggtcatgagcgagctggggggcgagcagtaggagtaggagcccagcggcagatccttgagcacctcgtggggcttccagcagaactcccggaagcctgggtggtccatgatcttgcgctcgatctcatggatcgtgaccaggcgctcactggtgaaaatgttgcgctccgcgtcgccgcgcgccaggaagatgagctcgatgcgccagtgcgcgtgcgtctgagtgttggcactcacataggcgcgcgagtagtcccagcgcgaggcgcctcggcgggcacggctctgattggccgcgactgccgcgtggggcgggatgctgggctggtaccgcccattcttgctcagccgctggtttcgcgggtcttcactctggttggctgccagatcctccaggggcggggtctcacgccgaagtcgcccgctccgattggctgtgggcttttgagccgcggaagtgtcccggtaagggcctgggccaccgagtgaggccgcggggatgacgcggggggctcgggaggcttgccgcgagcggttgccgagatgcagctgctgcagctgctctgagataaggcgctgaagcgtctcggaggtgaagtcggccaaatcgcgccggttccgcccccaggatccaaactgggacttaagcgccagagtgagagcgtcgaaacgctgtgaggcctcgtggttgcggatctcaaaggcgttgtaggagatgtcaatgtccagcggtgggtagtaaaggaacatgaaggctgacagggccatggggatgctgcagcccaggaagagcaccagcccagcacagcacggattggtgaaggcccagcccagggtactccagaagcccgaagctgggggtcgggaagccaggggccagtgccgccagcaacactgtccccctgccccaggttggggccctggcttctgggcccctaaaaaggtttcacccgttgcttcttcctcctcctgctcctcctctagccacacatcctgcagcaaggggtcatcctccgtgtccatagtctcggccggccgaacggggctaggctgagccgccggcgcgggagagagtgcgcagagggtcggggggcggcggccaccacgctgcgcagactcgtctcctcgcggaagtcgcagggggaagcttctcggagccgcaggaggctggggctccccctccgctccagggcaagcagaccgcgggaagctgcgcgcgaatcccagtcctcagctcgcaaccc

SEQ ID NO: 19091 - RNA, 164 nt, Homo sapiens
  source 1..164: mol_type = other RNA
tgggctgagggcaggaggcctgtgtggggagccaccgtgtcgggggagccgccgtgtagcgggggagctgctgtgtgagggggagccaccgtgtggggggaaccatggtgtgtggggggggagctgtcgtgtgcagggaagccacagtatggggggagccgtcg

SEQ ID NO: 19092 - RNA, 33 nt, Homo sapiens
  source 1..33: mol_type = other RNA
tggggacgtagctggccagacaggtgaccccag

SEQ ID NO: 19093 - RNA, 1001 nt, Homo sapiens
  source 1..1001: mol_type = other RNA
tggggagcggcccccgggtgggcatagtgggggagcccttgctgggagttgtggatgctgcccagaccggagctggagaggggcgagaggctctggcccatgccggccacgtccttgtggtagggggtatagaggttattcatggaggccagcccgcgctcatcccgcatgagcgtgaagctaccgctcacgttgcccgccaggcgctggtggtggtgcgggtggtggtggtgatggtggtggtggtgatggtgggggaacttgtccgagactgtggagatgggaggcagcggctgcagaggggtcaaggtggtgtaggtggtgggcatgctcatacctgggggagtctcgcaggccatggtcatggtgggatgcagggggccggccaggctgtgctcaggggcccggtggtggtggtggtaatctccgccgccgctgccgccgtccagcagggacgccatgcccatggagcgcgggtgcgcggggggcaggtggctgccgcggtgcgccacggagctgcgcgcgtgggggctgccgcccagcaggtcggcaggggcgggcaccggctcatggctcaccccgtgcagctcgccgatcgcttccatggtcagctgcgcgttcatcgtgatccgggcgagcaggcggcggacacaacatcgatgtggccaggcagaggcggcgaggggcgcacggagtccggtcttcacatcggctgctggcgactgttgccttccttcctctcactgtggggctctgtctctctctctctctctctccgtgtgtgtgtgtccgtgtgtgcgtgtgcgtgtgtgtgtgtgtgtgtgtctcgccttccctcttaccccccaccttcccctctgcgtcctcggcttttttttttttaatattaatttccaaagaggatccgcgccgttgggagagcgcagtgccccagcccgcccgcctcggccacctctcgcccctctctttcttaaaattctgaggtctccggctcccctgcc

SEQ ID NO: 19094 - RNA, 1003 nt, Homo sapiens
  source 1..1003: mol_type = other RNA
tggggagcggcccccgggtgggcatagtgggggagcccttgctgggagttgtggatgctgcccagaccggagctggagaggggcgagaggctctggcccatgccggccacgtccttgtggtagggggtatagaggttattcatggaggccagcccgcgctcatcccgcatgagcgtgaagctaccgctcacgttgcccgccaggcgctggtggtggtgcgggtggtggtggtgatggtggtggtggtgatggtgggggaacttgtccgagactgtggagatgggaggcagcggctgcagaggggtcaaggtggtgtaggtggtgggcatgctcatacctgggggagtctcgcaggccatggtcatggtgggatgcagggggccggccaggctgtgctcaggggcccggtggtggtggtggtaatctccgccgccgctgccgccgtccagcagggacgccatgcccatggagcgcgggtgcgcggggggcaggtggctgccgcggtgcgccacggagctgcgcgcgtgggggctgccgcccagcaggtcggcaggggcgggcaccggctcatggctcaccccgtgcagctcgccgatcgcttccatggtcagctgcgcgttcatcgtgatccgggcgagcaggcggcggacacaacatcgatgtggccaggcagaggcggcgaggggcgcacggagtccggtcttcacatcggctgctggcgactgttgccttccttcctctcactgtggggctctgtctctctctctctctctctccgtgtgtgtgtgtccgtgtgtgcgtgtgcgtgtgtgtgtgtgtgtgtgtctcgccttccctcttaccccccaccttcccctctgcgtcctcggcttttttttttttaatattaatttccaaagaggatccgcgccgttgggagagcgcagtgccccagcccgcccgcctcggccacctctcgcccctctctttcttaaaattctgaggtctccggctcccctgccgc

SEQ ID NO: 19095 - RNA, 1075 nt, Homo sapiens
  source 1..1075: mol_type = other RNA
tggggagcggcccccgggtgggcatagtgggggagcccttgctgggagttgtggatgctgcccagaccggagctggagaggggcgagaggctctggcccatgccggccacgtccttgtggtagggggtatagaggttattcatggaggccagcccgcgctcatcccgcatgagcgtgaagctaccgctcacgttgcccgccaggcgctggtggtggtgcgggtggtggtggtgatggtggtggtggtgatggtgggggaacttgtccgagactgtggagatgggaggcagcggctgcagaggggtcaaggtggtgtaggtggtgggcatgctcatacctgggggagtctcgcaggccatggtcatggtgggatgcagggggccggccaggctgtgctcaggggcccggtggtggtggtggtaatctccgccgccgctgccgccgtccagcagggacgccatgcccatggagcgcgggtgcgcggggggcaggtggctgccgcggtgcgccacggagctgcgcgcgtgggggctgccgcccagcaggtcggcaggggcgggcaccggctcatggctcaccccgtgcagctcgccgatcgcttccatggtcagctgcgcgttcatcgtgatccgggcgagcaggcggcggacacaacatcgatgtggccaggcagaggcggcgaggggcgcacggagtccggtcttcacatcggctgctggcgactgttgccttccttcctctcactgtggggctctgtctctctctctctctctctccgtgtgtgtgtgtccgtgtgtgcgtgtgcgtgtgtgtgtgtgtgtgtgtctcgccttccctcttaccccccaccttcccctctgcgtcctcggcttttttttttttaatattaatttccaaagaggatccgcgccgttgggagagcgcagtgccccagcccgcccgcctcggccacctctcgcccctctctttcttaaaattctgaggtctccggctcccctgccgcggcccgcgcgcctgccgcgtctgctgcctgcccgccccgctggccagcttgagccatggctctgttactgtt

SEQ ID NO: 19096 - RNA, 1494 nt, Homo sapiens
  source 1..1494: mol_type = other RNA
tggggagctgaggctctgggggtggagcccaacaatctctaaaacaagtcctccaggtgattgtaatgtacgctgtagcttgtaaaccactgccttagagctgttggaggattaagtgatgtttaatctacacatggctcaatgccagagaaattcagcatttaaaaaatttccttagaagtttctttttcttttccttcaagaattgttgaggataggaggaggtcatattgagagtttgtcatctcgtagaataatcagtatgagattagaaaaggtagaggttttttggattagaggcagtttagaaattgtgtgactggcttattattaatcgaattagcagtttctgtttcctggtttccccatcatttcacctgctactcagccgtaaaagtttatttttgattcaaatgcagagattgagttttgaaacaaatctagattagtaaacatctatacttatatatagatttataaaatataaccagattatctaaaacttataaatgcatcttaaaattttttctttcttttacaggcaggaatttatacgtgcatgtttaaaggcgatacttttcaaatgccagacttcctcagcttgtgctatacttcccgttcacacactgccgtgtctttgctatgccctcccatacaccaaaaaaaaaaaaaaaaaaaaaaaaacccaaataatccaaaaactcttgttcagatttccaaactggttcaaggtcaagatggaccaaaatttactttggctttatgttaaccaaagtcttcccaatcagtttcctaatatgtaaatgacatttttggtaaaagatgagcaaacatttcagaaatgagccaacaatttttttcttatccccatcataacttttaactgcaaaacctcaggacctggttcttttccaggctctgctgtctccatatagctgtgagtgtttttggtacaccaacacatctctgtatctgggccagtaaacttttttttttttttttttggtgtagggccaagcctacaatgcatatgtccttattgttcatctgttgtaactttttccacaaaaagtgtgtgaaatttagattgtggacgttccagtctccacttctgagccttgagaggttgctgaaagccctgactggctccagaaatgggcagtgttacctcttcagtgggtttcagtagctgtaaacttgaaacttaaggatttagtattgttctgaatgtggaattcacctccactgcaacttggatcctgtttaacaactcctcccttctctatattacctccatccatgtctgttcttatttgtaccctgaccctcaaaagttgcgtgacaaaagcatcaccttttgactgcagaaggcctgtttctttagtgcgtttagataagcctagtatcaggtgtgtaccattaccaaatacttgaggtgttaaggattaccatcttagcgttcatcctaccatttttatattcttaaggacaatt

SEQ ID NO: 19097 - RNA, 2370 nt, Homo sapiens
  source 1..2370: mol_type = other RNA
tggggcggagcttccggagccggtgagtacgggccgccttggacagcccctcgtggcggaacggtccactgggcacggccaccggcagctcgggggtcatgccgttgaggtcagcctgctcaaaggctgaagccccggctccaccgtctgggtccaccagctcctccgtggacgacatggtaccactggatgacgtccgctcgaacttcttaaagtcccctgcgccagggccggggtccagcccactgtccgagtctgagatcgagagcggccatgacttgtgaacctggtgtcctcgcccggccctgtggtccttggcaggtgtgccctcagtgcacccgccttcttctggggggctcccggcagcctccggccgcgccacatcactcacgttgaagctgctcttccgggcacgcatgacgggggaccaggcgttggcggagacgtggggctcaaagtcgtagtgcacatcgggctcctggtcccgctgcagctggcgcacgtgggaggcgtactgctggcctgggtcatacagcttgctgctctcacacagcatctggaagtgcacgggcagcggcgccgtctgcatatgcatcatctggtagtaggagatcgtggccgacttgatggtttggtcgctctgccggatgacctcctggatctgccgcagcgccgtcaccttggtatcctccagctcctgcttctgcgtcttcgcgtcggccacgcaggtgcggtaggtggccatagcttcctccgccttgttcttggcctcctcctccagccgccgccgcttgtccagggtcttggtggccgtgctgcctgctcccggcgcgctgccagcctgctcctcctccgccttggccacgaggaagcgagccttgtcgtggtcctcgcagcgctgcacgtaaccctgcttggccttgcgcaggttggactccgcctcttgcagcttcctctgggcacggtgccaggcctccttgatctccttcctgcgcttctcgtgttcaagccgccgcagggtcaggggctgcatgaaggtctgggtctgcaaggtgcccaccgcctgcaccatgctgtggccgaactccaggtcctgctccagggccagcgagtagatggacaggagcggcatgtggggctcctgcatgacgctctgtctgcagttgtgagcgatcttctgcaggcccttggcaaactccatctccagcgtcgtccgcttctccaggtagctgatgaggtccttcatgtacttggccatgttcttggcatacagcagtgcggcatccacgcccccctcacagcgctgtagcagcacgtccacctcctcggcgggcaggcagccggcgtcacagtcttccaggctgggaggcgtgccctcactgcccggtccatacaggctttccatggactggctcgagtccccaggaggcactgctaggagggtgctgctgtccacttcacccatgaggaactcggacactgtgctactgaaggccacagcaatcgtctccagggccttctcgaactcctgtttctccagatcattgttgctctcataatggaaggctttgaccttggcaatgagggtgccggctgcggtgagcgtctccacggtgttcagcagcgggtacttggagatgatctgatgcatgacacgcagagcctcacccaggcactcgtgggcccgcgggcggcgggcctcaaggaggtcgtcacgcaacacacactccttaagtttctcaaggccctcagcgaagcgggccacgtccgccagcagatgggagatgtcctcgacgacgtccgggccggcaccctcggtgggcagctcgcccgggctggcggctgtcagtgggctccggtggctccggcccagtgtccaggaggcagcacccgacagggggaagccagccgcgctggcgtggcggctcaggctggtgggccgcttgagggtccctgtggccttgacgccggaggacccagcgggcggctccaggcttggtccggggaacaccgcgtcagccccatccttcctgggcagctcccccgagggctgcgggctggggcttcccgcgcggttctttttcgagatggaaggggttttcatgagctctcgtttcttcctggagaacatgatggggccccggccgggagcccgagggggcgggctgggggtctcagcgctgcagctcccggcgctggccgcttcgggaccacattgtcgccggccaccccctccccagctgtcaggcccacgtgacaggcccggccgtcactggcgggccctccccccaacaggaaaaggcttcggggaggcggcgacgcggcctcgcccccgacccttcccggcctcagcctgcggctctgcggagt

SEQ ID NO: 19098 - RNA, 2218 nt, Homo sapiens
  source 1..2218: mol_type = other RNA
tggggcggagcttccggagccggtgagtacgggccgccttggacagcccctcgtggcggaacggtccactgggcacggccaccggcagctcgggggtcatgccgttgaggtcagcctgctcaaaggctgaagccccggctccaccgtctgggtccaccagctcctccgtggacgacatggtaccactggatgacgtccgctcgaacttcttaaagtcccctgcgccagggccggggtccagcccactgtccgagtctgagatcgagagcggccatgacttgtgaacctggtgtcctcgcccggccctgtggtccttggcaggtgtgccctcagtgcacccgccttcttctggggggctcccggcagcctccggccgcgccacatcactcacgttgaagctgctcttccgggcacgcatgacgggggaccaggcgttggcggagacgtggggctcaaagtcgtagtgcacatcgggctcctggtcccgctgcagctggcgcacgtgggaggcgtactgctggcctgggtcatacagcttgctgctctcacacagcatctggaagtgcacgggcagcggcgccgtctgcatatgcatcatctggtagtaggagatcgtggccgacttgatggtttggtcgctctgccggatgacctcctggatctgccgcagcgccgtcaccttggtatcctccagctcctgcttctgcgtcttcgcgtcggccacgcaggtgcggtaggtggccatagcttcctccgccttgttcttggcctcctcctccagccgccgccgcttgtccagggtcttggtggccgtgctgcctgctcccggcgcgctgccagcctgctcctcctccgccttggccacgaggaagcgagccttgtcgtggtcctcgcagcgctgcacgtaaccctgcttggccttgcgcaggttggactccgcctcttgcagcttcctctgggcacggtgccaggcctccttgatctccttcctgcgcttctcgtgttcaagccgccgcagggtcaggggctgcatgaaggtctgggtctgcaaggtgcccaccgcctgcaccatgctgtggccgaactccaggtcctgctccagggccagcgagtagatggacaggagcggcatgtggggctcctgcatgacgctctgtctgcagttgtgagcgatcttctgcaggcccttggcaaactccatctccagcgtcgtccgcttctccaggtagctgatgaggtccttcatgtacttggccatgttcttggcatacagcagtgcggcatccacgcccccctcacagcgctgtagcagcacgtccacctcctcggcgggcaggcagccggcgtcacagtcttccaggctgggaggcgtgccctcactgcccggtccatacaggctttccatggactggctcgagtccccaggaggcactgctaggagggtgctgctgtccacttcacccatgaggaactcggacactgtgctactgaaggccacagcaatcgtctccagggccttctcgaactcctgtttctccagatcattgttgctctcataatggaaggctttgaccttggcaatgagggtgccggctgcggtgagcgtctccacggtgttcagcagcgggtacttggagatgatctgatgcatgacacgcagagcctcacccaggcactcgtgggcccgcgggcggcgggcctcaaggaggtcgtcacgcaacacacactccttaagtttctcaaggccctcagcgaagcgggccacgtccgccagcagatgggagatgtcctcgacgacgtccgggccggcaccctcggtgggcagctcgcccgggctggcggctgtcagtgggctccggtggctccggcccagtgtccaggaggcagcacccgacagggggaagccagccgcgctggcgtggcggctcaggctggtgggccgcttgagggtccctgtggccttgacgccggaggacccagcgggcggctccaggcttggtccggggaacaccgcgtcagccccatccttcctgggcagctccgtgagctgaatgccggggtcccggcctctctgctgtggcccctgccgtcccgcccggtaggggctgtagctggcacgagcccccagccgccgccccagcatgagccccgagcacagggcgggtccctgtccccctgcggcccggcgtcagctccgggtctcacccgggctccactc

SEQ ID NO: 19099 - RNA, 2246 nt, Homo sapiens
  source 1..2246: mol_type = other RNA
tggggcggagcttccggagccggtgagtacgggccgccttggacagcccctcgtggcggaacggtccactgggcacggccaccggcagctcgggggtcatgccgttgaggtcagcctgctcaaaggctgaagccccggctccaccgtctgggtccaccagctcctccgtggacgacatggtaccactggatgacgtccgctcgaacttcttaaagtcccctgcgccagggccggggtccagcccactgtccgagtctgagatcgagagcggccatgacttgtgaacctggtgtcctcgcccggccctgtggtccttggcaggtgtgccctcagtgcacccgccttcttctggggggctcccggcagcctccggccgcgccacatcactcacgttgaagctgctcttccgggcacgcatgacgggggaccaggcgttggcggagacgtggggctcaaagtcgtagtgcacatcgggctcctggtcccgctgcagctggcgcacgtgggaggcgtactgctggcctgggtcatacagcttgctgctctcacacagcatctggaagtgcacgggcagcggcgccgtctgcatatgcatcatctggtagtaggagatcgtggccgacttgatggtttggtcgctctgccggatgacctcctggatctgccgcagcgccgtcaccttggtatcctccagctcctgcttctgcgtcttcgcgtcggccacgcaggtgcggtaggtggccatagcttcctccgccttgttcttggcctcctcctccagccgccgccgcttgtccagggtcttggtggccgtgctgcctgctcccggcgcgctgccagcctgctcctcctccgccttggccacgaggaagcgagccttgtcgtggtcctcgcagcgctgcacgtaaccctgcttggccttgcgcaggttggactccgcctcttgcagcttcctctgggcacggtgccaggcctccttgatctccttcctgcgcttctcgtgttcaagccgccgcagggtcaggggctgcatgaaggtctgggtctgcaaggtgcccaccgcctgcaccatgctgtggccgaactccaggtcctgctccagggccagcgagtagatggacaggagcggcatgtggggctcctgcatgacgctctgtctgcagttgtgagcgatcttctgcaggcccttggcaaactccatctccagcgtcgtccgcttctccaggtagctgatgaggtccttcatgtacttggccatgttcttggcatacagcagtgcggcatccacgcccccctcacagcgctgtagcagcacgtccacctcctcggcgggcaggcagccggcgtcacagtcttccaggctgggaggcgtgccctcactgcccggtccatacaggctttccatggactggctcgagtccccaggaggcactgctaggagggtgctgctgtccacttcacccatgaggaactcggacactgtgctactgaaggccacagcaatcgtctccagggccttctcgaactcctgtttctccagatcattgttgctctcataatggaaggctttgaccttggcaatgagggtgccggctgcggtgagcgtctccacggtgttcagcagcgggtacttggagatgatctgatgcatgacacgcagagcctcacccaggcactcgtgggcccgcgggcggcgggcctcaaggaggtcgtcacgcaacacacactccttaagtttctcaaggccctcagcgaagcgggccacgtccgccagcagatgggagatgtcctcgacgacgtccgggccggcaccctcggtgggcagctcgcccgggctggcggctgtcagtgggctccggtggctccggcccagtgtccaggaggcagcacccgacagggggaagccagccgcgctggcgtggcggctcaggctggtgggccgcttgagggtccctgtggccttgacgccggaggacccagcgggcggctccaggcttggtccggggaacaccgcgtcagccccatccttcctgggcagctcctcgggtgggaggggcagatctctggggcacaggacatgaaggccacagccccttgctccaagtctggctctccaggcccaggtccaagtgcaaacccagcccagcagacccttgagaactctttgcccccgactcatggcgctgagggctggggtcagagggtgagggtcagctggatgtcggatgggcttctggcccggccct

SEQ ID NO: 19100 - RNA, 1859 nt, Homo sapiens
  source 1..1859: mol_type = other RNA
tggggcggagcttccggagccggtgagtacgggccgccttggacagcccctcgtggcggaacggtccactgggcacggccaccggcagctcgggggtcatgccgttgaggtcagcctgctcaaaggctgaagccccggctccaccgtctgggtccaccagctcctccgtggacgacatggtaccactggatgacgtccgctcgaacttcttaaagtcccctgcgccagggccggggtccagcccactgtccgagtctgagatcgagagcggccatgacttgtgaacctggtgtcctcgcccggccctgtggtccttggcaggtgtgccctcagtgcacccgccttcttctggggggctcccggcagcctccggccgcgccacatcactcacgttgaagctgctcttccgggcacgcatgacgggggaccaggcgttggcggagacgtggggctcaaagtcgtagtgcacatcgggctcctggtcccgctgcagctggcgcacgtgggaggcgtactgctggcctgggtcatacagcttgctgctctcacacagcatctggaagtgcacgggcagcggcgccgtctgcatatgcatcatctggtagtaggagatcgtggccgacttgatggtttggtcgctctgccggatgacctcctggatctgccgcagcgccgtcaccttggtatcctccagctcctgcttctgcgtcttcgcgtcggccacgcaggtgcggtaggtggccatagcttcctccgccttgttcttggcctcctcctccagccgccgccgcttgtccagggtcttggtggccgtgctgcctgctcccggcgcgctgccagcctgctcctcctccgccttggccacgaggaagcgagccttgtcgtggtcctcgcagcgctgcacgtaaccctgcttggccttgcgcaggttggactccgcctcttgcagcttcctctgggcacggtgccaggcctccttgatctccttcctgcgcttctcgtgttcaagccgccgcagggtcaggggctgcatgaaggtctgggtctgcaaggtgcccaccgcctgcaccatgctgtggccgaactccaggtcctgctccagggccagcgagtagatggacaggagcggcatgtggggctcctgcatgacgctctgtctgcagttgtgagcgatcttctgcaggcccttggcaaactccatctccagcgtcgtccgcttctccaggtagctgatgaggtccttcatgtacttggccatgttcttggcatacagcagtgcggcatccacgcccccctcacagcgctgtagcagcacgtccacctcctcggcgggcaggcagccggcgtcacagtcttccaggctgggaggcgtgccctcactgcccggtccatacaggctttccatggactggctcgagtccccaggaggcactgctaggagggtgctgctgtccacttcacccatgaggaactcggacactgtgctactgaaggccacagcaatcgtctccagggccttctcgaactcctgtttctccagatcattgttgctctcataatggaaggctttgaccttggcaatgagggtgccggctgcggtgagcgtctccacggtgttcagcagcgggtacttggagatgatctgatgcatgacacgcagagcctcacccaggcactcgtgggcccgcgggcggcgggcctcaaggaggtctcgggggcccgcccggcagcgcacggggccctcgtccagcaccgggtgcgccgtcccgcagatacacatggcgcagccgtcggggcgcggagaccgcgagcgcgtggggcctggcagctgaccgatgggggtctccggtggccaaacc

SEQ ID NO: 19101 - RNA, 1407 nt, Homo sapiens
  source 1..1407: mol_type = other RNA
tggggcggagcttccggagccggtgagtacgggccgccttggacagcccctcgtggcggaacggtccactgggcacggccaccggcagctcgggggtcatgccgttgaggtcagcctgctcaaaggctgaagccccggctccaccgtctgggtccaccagctcctccgtggacgacatggtaccactggatgacgtccgctcgaacttcttaaagtcccctgcgccagggccggggtccagcccactgtccgagtctgagatcgagagcggccatgacttgtgaacctggtgtcctcgcccggccctgtggtccttggcaggtgtgccctcagtgcacccgccttcttctggggggctcccggcagcctccggccgcgccacatcactcacgttgaagctgctcttccgggcacgcatgacgggggaccaggcgttggcggagacgtggggctcaaagtcgtagtgcacatcgggctcctggtcccgctgcagctggcgcacgtgggaggcgtactgctggcctgggtcatacagcttgctgctctcacacagcatctggaagtgcacgggcagcggcgccgtctgcatatgcatcatctggtagtaggagatcgtggccgacttgatggtttggtcgctctgccggatgacctcctggatctgccgcagcgccgtcaccttggtatcctccagctcctgcttctgcgtcttcgcgtcggccacgcaggtgcggtaggtggccatagcttcctccgccttgttcttggcctcctcctccagccgccgccgcttgtccagggtcttggtggccgtgctgcctgctcccggcgcgctgccagcctgctcctcctccgccttggccacgaggaagcgagccttgtcgtggtcctcgcagcgctgcacgtaaccctgcttggccttgcgcaggttggactccgcctcttgctgtgggtgtgggagccaggaggccagttccaaccctatcctcggatgggactcagtctccccagctcctcctttcctccccacccccatctctctcagcaaggccccatggcccagctgggcatgcagaggaccctgcacaacaatcggcagcggaaaaacaggaggagtggccgggcgcggtggctcacgtctgtaatcccagcactttgggaggccgaggcaggtggatcacttgaggtcaggagtttgagaccagcctggccaacatagtgaaaccccgtatctacccaaaatttaaaacaattagccgggcattgtggtgcacgcttgtaatcccagctactcgggaggctgaggcactagaatcgcgaacagcttgaacccaggaggcgaaggttgcagtgagccaagattgcatgcaccactgcactccagcctgggcaacagagattccagct

SEQ ID NO: 19102 - RNA, 1276 nt, Homo sapiens
  source 1..1276: mol_type = other RNA
tggggcggagcttccggagccggtgagtacgggccgccttggacagcccctcgtggcggaacggtccactgggcacggccaccggcagctcgggggtcatgccgttgaggtcagcctgctcaaaggctgaagccccggctccaccgtctgggtccaccagctcctccgtggacgacatggtaccactggatgacgtccgctcgaacttcttaaagtcccctgcgccagggccggggtccagcccactgtccgagtctgagatcgagagcggccatgacttgtgaacctggtgtcctcgcccggctggagaaagaggcgtctctggtgaagggccagggtgggtcgcagggagccagcgtccgcccctgggccccgccggacactcacccctgtggtccttggcaggtgtgccctcagtgcacccgccttcttctggggggctcccggcagcctccggccgcgccacatcactcacgttgaagctgctcttccgggcacgcatgacgggggaccaggcgttggcggagacgtggggctcaaagtcgtagtgcacatcgggctcctggtcccgctgcagctggcgcacgtgggaggcgtactgctggcctgggtcatacagcttgctgctctcacacagcatctggaagtgcacgggcagcggcgccgtctgcatatgcatcatctggtagtaggagatcgtggccgacttgatggtttggtcgctctgccggatgacctcctggatctgccgcagcgccgtcaccttggtatcctccagctcctgcttctgcgtcttcgcgtcggccacgcaggtgcggtaggtggccatagcttcctccgccttgttcttggcctcctcctccagccgccgccgcttgtccagggtcttggtggccgtgctgcctgctcccggcgcgctgccagcctgctcctcctccgccttggccacgaggaagcgagccttgtcgtggtcctcgcagcgctgcacgtaaccctgcttggccttgcgcaggttggactccgcctcttgaaccgagggaggcacggcttctccccatttctgcagggacagcagtgagcgccgggctcctgggtccttccaggcagagctgggggcgacggggctggagcatctccgacccggcttggcgttggggggggcggcccagcctgcgaggccgcgcatgcgcaggaggccggggcgtgtgcggagctcgccgcagggccctcgctatggggctggggctgggactgcgcctgcgccgaggcccgctgc

SEQ ID NO: 19103 - RNA, 2454 nt, Homo sapiens
  source 1..2454: mol_type = other RNA
tggggcggagcttccggagccggtgagtacgggccgccttggacagcccctcgtggcggaacggtccactgggcacggccaccggcagctcgggggtcatgccgttgaggtcagcctgctcaaaggctgaagccccggctccaccgtctgggtccaccagctcctccgtggacgacatggtaccactggatgacgtccgctcgaacttcttaaagtcccctgcgccagggccggggtccagcccactgtccgagtctgagatcgagagcggccatgacttgtgaacctggtgtcctcgcccggctggagaaagaggcgtctctggtgaagggccagggtgggtcgcagggagccagcgtccgcccctgggccccgccggacactcacccctgtggtccttggcaggtgtgccctcagtgcacccgccttcttctggggggctcccggcagcctccggccgcgccacatcactcacgttgaagctgctcttccgggcacgcatgacgggggaccaggcgttggcggagacgtggggctcaaagtcgtagtgcacatcgggctcctggtcccgctgcagctggcgcacgtgggaggcgtactgctggcctgggtcatacagcttgctgctctcacacagcatctggaagtgcacgggcagcggcgccgtctgcatatgcatcatctggtagtaggagatcgtggccgacttgatggtttggtcgctctgccggatgacctcctggatctgccgcagcgccgtcaccttggtatcctccagctcctgcttctgcgtcttcgcgtcggccacgcaggtgcggtaggtggccatagcttcctccgccttgttcttggcctcctcctccagccgccgccgcttgtccagggtcttggtggccgtgctgcctgctcccggcgcgctgccagcctgctcctcctccgccttggccacgaggaagcgagccttgtcgtggtcctcgcagcgctgcacgtaaccctgcttggccttgcgcaggttggactccgcctcttgcagcttcctctgggcacggtgccaggcctccttgatctccttcctgcgcttctcgtgttcaagccgccgcagggtcaggggctgcatgaaggtctgggtctgcaaggtgcccaccgcctgcaccatgctgtggccgaactccaggtcctgctccagggccagcgagtagatggacaggagcggcatgtggggctcctgcatgacgctctgtctgcagttgtgagcgatcttctgcaggcccttggcaaactccatctccagcgtcgtccgcttctccaggtagctgatgaggtccttcatgtacttggccatgttcttggcatacagcagtgcggcatccacgcccccctcacagcgctgtagcagcacgtccacctcctcggcgggcaggcagccggcgtcacagtcttccaggctgggaggcgtgccctcactgcccggtccatacaggctttccatggactggctcgagtccccaggaggcactgctaggagggtgctgctgtccacttcacccatgaggaactcggacactgtgctactgaaggccacagcaatcgtctccagggccttctcgaactcctgtttctccagatcattgttgctctcataatggaaggctttgaccttggcaatgagggtgccggctgcggtgagcgtctccacggtgttcagcagcgggtacttggagatgatctgatgcatgacacgcagagcctcacccaggcactcgtgggcccgcgggcggcgggcctcaaggaggtcgtcacgcaacacacactccttaagtttctcaaggccctcagcgaagcgggccacgtccgccagcagatgggagatgtcctcgacgacgtccgggccggcaccctcggtgggcagctcgcccgggctggcggctgtcagtgggctccggtggctccggcccagtgtccaggaggcagcacccgacagggggaagccagccgcgctggcgtggcggctcaggctggtgggccgcttgagggtccctgtggccttgacgccggaggacccagcgggcggctccaggcttggtccggggaacaccgcgtcagccccatccttcctgggcagctcccccgagggctgcgggctggggcttcccgcgcggttctttttcgagatggaaggggttttcatgagctctcgtttcttcctggagaacatgatggggccccggccgggagcccgagggggcgggctgggggtctcagcgctgcagctcccggcgctggccgcttcgggaccacattgtcgccggccaccccctccccagctgtcaggcccacgtgacaggcccggccgtcactggcgggccctccccccaacaggaaaaggcttcggggaggcggcgacgcggcctcgcccccgacccttcccggcctcagcctgcggctctgcggagt

SEQ ID NO: 19104 - RNA, 2302 nt, Homo sapiens
  source 1..2302: mol_type = other RNA
tggggcggagcttccggagccggtgagtacgggccgccttggacagcccctcgtggcggaacggtccactgggcacggccaccggcagctcgggggtcatgccgttgaggtcagcctgctcaaaggctgaagccccggctccaccgtctgggtccaccagctcctccgtggacgacatggtaccactggatgacgtccgctcgaacttcttaaagtcccctgcgccagggccggggtccagcccactgtccgagtctgagatcgagagcggccatgacttgtgaacctggtgtcctcgcccggctggagaaagaggcgtctctggtgaagggccagggtgggtcgcagggagccagcgtccgcccctgggccccgccggacactcacccctgtggtccttggcaggtgtgccctcagtgcacccgccttcttctggggggctcccggcagcctccggccgcgccacatcactcacgttgaagctgctcttccgggcacgcatgacgggggaccaggcgttggcggagacgtggggctcaaagtcgtagtgcacatcgggctcctggtcccgctgcagctggcgcacgtgggaggcgtactgctggcctgggtcatacagcttgctgctctcacacagcatctggaagtgcacgggcagcggcgccgtctgcatatgcatcatctggtagtaggagatcgtggccgacttgatggtttggtcgctctgccggatgacctcctggatctgccgcagcgccgtcaccttggtatcctccagctcctgcttctgcgtcttcgcgtcggccacgcaggtgcggtaggtggccatagcttcctccgccttgttcttggcctcctcctccagccgccgccgcttgtccagggtcttggtggccgtgctgcctgctcccggcgcgctgccagcctgctcctcctccgccttggccacgaggaagcgagccttgtcgtggtcctcgcagcgctgcacgtaaccctgcttggccttgcgcaggttggactccgcctcttgcagcttcctctgggcacggtgccaggcctccttgatctccttcctgcgcttctcgtgttcaagccgccgcagggtcaggggctgcatgaaggtctgggtctgcaaggtgcccaccgcctgcaccatgctgtggccgaactccaggtcctgctccagggccagcgagtagatggacaggagcggcatgtggggctcctgcatgacgctctgtctgcagttgtgagcgatcttctgcaggcccttggcaaactccatctccagcgtcgtccgcttctccaggtagctgatgaggtccttcatgtacttggccatgttcttggcatacagcagtgcggcatccacgcccccctcacagcgctgtagcagcacgtccacctcctcggcgggcaggcagccggcgtcacagtcttccaggctgggaggcgtgccctcactgcccggtccatacaggctttccatggactggctcgagtccccaggaggcactgctaggagggtgctgctgtccacttcacccatgaggaactcggacactgtgctactgaaggccacagcaatcgtctccagggccttctcgaactcctgtttctccagatcattgttgctctcataatggaaggctttgaccttggcaatgagggtgccggctgcggtgagcgtctccacggtgttcagcagcgggtacttggagatgatctgatgcatgacacgcagagcctcacccaggcactcgtgggcccgcgggcggcgggcctcaaggaggtcgtcacgcaacacacactccttaagtttctcaaggccctcagcgaagcgggccacgtccgccagcagatgggagatgtcctcgacgacgtccgggccggcaccctcggtgggcagctcgcccgggctggcggctgtcagtgggctccggtggctccggcccagtgtccaggaggcagcacccgacagggggaagccagccgcgctggcgtggcggctcaggctggtgggccgcttgagggtccctgtggccttgacgccggaggacccagcgggcggctccaggcttggtccggggaacaccgcgtcagccccatccttcctgggcagctccgtgagctgaatgccggggtcccggcctctctgctgtggcccctgccgtcccgcccggtaggggctgtagctggcacgagcccccagccgccgccccagcatgagccccgagcacagggcgggtccctgtccccctgcggcccggcgtcagctccgggtctcacccgggctccactc

SEQ ID NO: 19105 - RNA, 1488 nt, Homo sapiens
  source 1..1488: mol_type = other RNA
tggggcggggcaggtccctgcggagaggcacttctggcctgaagacagctccattgagcccctgcagtacaggcgtagtgccttggaccaagcccacagcctggtaaggggcgcctgccagggccacggccaggaggcattccccgaagccttgctcccctggtgcagcagggctgtgggaggtggtgacattgaggccagcctctttcaccagcagcttagcgttcaccaagttcacatccgcctgcttggaagcctctttcaggaggccgacaatgactgcggggcttaggcagttcccagcattcttcagggatgttccctgtgttatcacctggatggtccctttgggggacccagcccaggctcgcatcagtgtccccagagcttctgccagaccaatccaaggcttggtgtgtggagagaaggcactggtaagggcctgggcattcacaacccccgtgagagatttccccttcaccatgtccacgaactgaacagcaatttcctccccacagcggctctgagcctccttggtgctggcacccaggtggggacagctgatgacattctcatggtccaccaaggcccggtcccgtggcggctcttccgtaaacacgtccagtgcagccccggcacactggccagactgcagggcccggagcagggcgccttcgtccacgatccctccacgggcacagttcaccacacgcacccccttcttgcactgggcaaaggtgttgtcattcagcaagcctgtcgtggagggcaggagaggagtgtgcacagtgatgaaatcacagagaggccagatctcctccaggggcagctgctgaacaccaaaggaggccgagacctctggggaaatgatggggtcataccctatagtcttcatcccaaaggactgcatccgggtagctacctctctcccaatcctgcccaggccaagaattcccagggtctttccattcagctctgttcccatgaacttcttccgctcccatttgccgtccttcatcgaagccgtcgcctggggaatctgcctggccaggcacatgatcattccacaagtgagttctgcggcactgaggctgttcccattgggggtgttcataaccaagatgcccttccttgttgcggcctccagatccacattgtccacacctgtgccagccctgcccaccacctggagtttctcagctgcgttgatgacatcagcggtcaccttggtggcagagcgaacaataaggccttcacagtcctgcagctccgctatcagctcctctttgctaaggttctgcttttccaccacctgcagccctccatcttgcaagatcttccggcagcaagggtccaggctgtcactgatgagcactttccgcagatttgcaaaagccattgctggagttggcctcggaatcggccgctgtgagtagaagtacctaagccaagaagctgcggttcggcctggcgcgctagagtaactgg

SEQ ID NO: 19106 - RNA, 1708 nt, Homo sapiens
  source 1..1708: mol_type = other RNA
tggggcggggcaggtccctgcggagaggcacttctggcctgaagacagctccattgagcccctgcagtacaggcgtagtgccttggaccaagcccacagcctggtaaggggcgcctgccagggccacggccaggaggcattccccgaagccttgctcccctggtgcagcagggctgtgggaggtggtgacattgaggccagcctctttcaccagcagcttagcgttcaccaagttcacatccgcctgcttggaagcctctttcaggaggccgacaatgactgcggggcttaggcagttcccagcattcttcagggatgttccctgtgttatcacctggatggtccctttgggggacccagcccaggctcgcatcagtgtccccagagcttctgccagaccaatccaaggcttggtgtgtggagagaaggcactggtaagggcctgggcattcacaacccccgtgagagatttccccttcaccatgtccacgaactgaacagcaatttcctccccacagcggctctgagcctccttggtgctggcacccaggtggggacagctgatgacattctcatggtccaccaaggcccggtcccgtggcggctcttccgtaaacacgtccagtgcagccccggcacactggccagactgcagggcccggagcagggcgccttcgtccacgatccctccacgggcacagttcaccacacgcacccccttcttgcactgggcaaaggtgttgtcattcagcaagcctgtcgtggagggcaggagaggagtgtgcacagtgatgaaatcacagagaggccagatctcctccaggggcagctgctgaacaccaaaggaggccgagacctctggggaaatgatggggtcataccctatagtcttcatcccaaaggactgcatccgggtagctacctctctcccaatcctgcccaggccaagaattcccagggtctttccattcagctctgttcccatgaacttcttccgctcccatttgccgtccttcatcgaagccgtcgcctggggaatctgcctttgatgagtgaggtcatggtgagcagttgacaatggggagcttcttttaaaccacagcatttcaccgattcctttaaacaaagctggtccagagagctcagatggaaactgcagggaggagttagagcagaggtaaattcccccagatcctcctccagcaggagggaaagcaggtctcgccatgggaaaagtaatttcttggtcccggaaggtttcaggcctggccaggcacatgatcattccacaagtgagttctgcggcactgaggctgttcccattgggggtgttcataaccaagatgcccttccttgttgcggcctccagatccacattgtccacacctgtgccagccctgcccaccacctggagtttctcagctgcgttgatgacatcagcggtcaccttggtggcagagcgaacaataaggccttcacagtcctgcagctccgctatcagctcctctttgctaaggttctgcttttccaccacctgcagccctccatcttgcaagatcttccggcagcaagggtccaggctgtcactgatgagcactttccgcagatttgcaaaagccattgctggagttggcctcggaatcggccgctgtgagtagaagtacctaagccaagaagctgcggttcggcctggcgcgctagagtaact

SEQ ID NO: 19107 - RNA, 6591 nt, Homo sapiens
  source 1..6591: mol_type = other RNA
tggggcggggcaggtccctgcggagaggcacttctggcctgaagacagctccattgagcccctgcagtacaggcgtagtgccttggaccaagcccacagcctggtaaggggcgcctgccagggccacggccaggaggcattccccgaagccttgctcccctggtgcagcagggctgtgggaggtggtgacattgaggccagcctctttcaccagcagcttagcgttcaccaagttcacatccgcctgcttggaagcctctttcaggaggccgacaatgactgcggggcttaggcagttcccagcattcttcagggatgttccctgtgttatcacctggatggtccctttgggggacccagcccaggctcgcatcagtgtccccagagcttctgccagaccaatccaaggcttggtgtgtggagagaaggcactggtaagggcctgggcattcacaacccccgtgagagatttccccttcaccatgtccacgaactgaacagcaatttcctccccacagcggctctgagcctccttggtgctggcacccaggtggggacagctgatgacattctcatggtccaccaaggcccggtcccgtggcggctcttccgtaaacacgtccagtgcagccccggcacactggccagactgcagggcccggagcagggcgccttcgtccacgatccctccacgggcacagttcaccacacgcacccccttcttgcactgggcaaaggtgttgtcattcagcaagcctgtcgtggagggcaggagaggagtgtgcacagtgatgaaatcacagagaggccagatctcctccaggggcagctgctgaacaccaaaggaggccgagacctctggggaaatgatggggtcataccctatagtcttcatcccaaaggactgcatccgggtagctacctctctcccaatcctgcccaggccaagaattcccagggtctttccattcagctctgttcccatgaacttcttccgctcccatttgccgtccttcatcgaagccgtcgcctggggaatctgcctttgatgagtgaggtcatggtgagcagttgacaatggggagcttcttttaaaccacagcatttcaccgattcctttaaacaaagctggtccagagagctcagatggaaactgcagggaggagttagagcagaggtaaattcccccagatcctcctccagcaggagggaaagcaggtctcgccatgggaaaagtaatttcttggtcccggaaggtttcaggcctggccaggcacatgatcattccacaagtgagttctgcggcactgaggctgttcccattgggggtgttcataaccaagatgcccttccttgttgcggcctccagatccacattgtccacacctgtgccagccctgcccaccacctggagtttctcagctgcgttgatgacatcagcggtcaccttggtggcagagcgaacaataaggccttcacagtcctgtaaaataaaagagatggagcacatggctcctcagatccattttccccgtagagctctcagctggatcccatgaaaaccttcttttaccttcattcccactgcatggattcagcagagagaaacatgcaggcggcctggaagacactccaaatccttttatgtctgaggttctgaagcagaacgtcagagtgggagatttgaagaaatgttcaccagcatctggtccaactccattttacagaggaaaaactgaagcccaacaaagttaagcctgcctactttcccttcccctcccctgtacttttcttccttcattttatcggatgcccgctatgtacgtatctggcattatgctaaactgattatgacctgggtgtatacaagtcacatgggcacccagggcttagaggaatcaaacagaagccacctcagtgctgactgccccagtgctgaggccaacaccaggtgagcacctggaggtattctgatttccccccatagcagcctagttaaatatcagccaagccaggcagaaacaggatactggcatcttttccacattcaagtccaccacacaggctccaaagaaaaggatttccctgcctggacacactttactgacttttcaaggtgcaataaagttatcttccaggaaacatttgccaacaaccctgaactgtcactctccctacaccccaccatttttgttgtgatcaccaatataatatgtttcatatctagttgtcctctcttagacctgcagttttggtctccttagttatattttctatgcctaatgcagggattttatattaaaactttatctactctataccatatatccatagtaccagcctcaccagcacataaaccatttattgagcacctgctgggtactaggcattacaccagttgctttacattattctcttcacaactccaaggagaaggggtataatcatccccagtttccagataaagaaacagaggctttgagaggtaacctgcccaaggtcactcttacagatcaaaaaccagccaagaactggaaagtcattgccactggctaactctgagactgtaactgaagaagagttggtagacctgccaagatgtcaagaagatagggccagagccaaggccatggccagttaggtgcaaaaaccaaactgtaaaatcccttggagagatttactagtaacaatagctaccattttttgagcaagtactttacatccagcactgtgcttcacaacaatcctaagacagatattacaattatccctatagtacagacaagcaaactgacacttaaagaatttagagaacttgctgaagtcacatagctaggatatggcagaagctggaatcaagtccaaatctgttgagttccaactaccttccaaatacagcatttagacacctaaaccaggagagacattgccagaaatcctgtggcttctccaagatggcagaagctccctaacaaaggtccctggatcttctggtgacctgctcctcccagccagcctgcctactgggggataatagaaataggcacaaatgcctctgtcgagaagagcaagttgcctgtggcctgtaggcaagctcacagttgatacttcacaatgaagtgttttatacacttccattgaataaatgaattcagtgatgagaggccggtagaaaccaccctcatcagtcccccatcctcacaccttcaccctctttcccaaataactttaacacttcacatgcctgaaaattgctcatcagaaatcccttcctttgactgtgataaggaggcataaggtctacttctaagagtgctcaaggattttcaaaaatcttattaaaagaagttgaaaaaaagcaggaaaaacgttcagaaattgacaaatcagtcaacagaactaaatagacactagacaaacagaatatgtgagaatttagaaaataaaaagcagaactcaaattgatgcggaaaggaagaactaaacaagaaataatgttatgaaaattcaagaagaaaaataatagattgctacctcacttcagatttttaaaaatccagatgaattaaagaatttttaaaaatataagcattaaaagaaaatgtcaggggatatttttatgactcggattgggaaaacctttcataagcaaggcacaaatcttagaaactctggaagaaaatattgacaaatccagttacattcaaattttaaacttctgcatggaaaaagatcccataaacaaaagcaagtagtggtcctgatatgtggagaaaactcctttcaccatatgtaacagaacaaggattcatcaccaaaagtgatagaattcctacaaatcaactttttttttttttttttttttttttttttgagacagagtttcactcttattgcccaggctggagtgcaatggcgcgatcttggctcactgcaacctccgcctcccgggttcaagcgattctcctgcttcagcctcccgagtagctgggattataggcatgcaccacaaatccacttttttaaaggataaagagcacaataaaaaatagataaatatataaataggcaatgcacagaagaactacaaagtggtcactagtttcactagtttatagactcttcaacgctagatatcaaggaaatatagatttttaaatatgatatttttgggcatcattttggcagaaagaaaatgaataatattcagcattggtgagcatggagggaaacaggagtgtacactgcatgacctttttggagggcaactgggcagtgggtgggtaagcacatttttagtggtcatttctttgcagccagcactgacaccttagaaaattggtaacacactgaggaaacacaacctcctttcaagtggtcagctcaggaccaaaagtcaaagttcaactgacaagaagcaggcatggagcaagaggagaagggaccacccagagtcatcatcttatcaccttgtctctctagcatcaagttccagagcccacatctcaggcccagtcctgctccagaggctctaccaatcactcccttgggccttaagggtccatccttcttcaatgttctctccaaagctgccaaaatgctccccaaaccttgcaaacctgctccccacaggcaacactagctggagagcatgcagactccccaaagtccacccattcttgtagcccctgaacaagcacagaaacagcactattgtttctttcatgagcatggactctctggatggatctcccttgtaaagatttatgctgtagtctcttcacttttccctcaaaccagccttctttggtgccagggaaactaagagtccccagtcagactcctacagatgagcatcaggtctcacctctcccaagggcagaaactgtcactcaggagaccttggtcccacattagaaccagacatcccacatcagtcagagttaatgagcttccaaggcctcttacaacctcaactacccactctatccactcattcaatcagcacatattcacagacagcctgaatccaacctacctcctgctggaccctcaaagcccctgcacccaagccccttccctcctcacgccacaacgcacccccttcaaagactttgccccaagctgtctgctcctgtcctctacttatggaaaccacagccctaaccaaatgcacccatctgctcacatcctctgcagtttgcgattaaaacttctccagtgtccagagatcctcccctctctttgtcattccttgggtgaggaagcaagtctctctctacacagcaccaaattctgatgttcactgccctctgcgtgtggcttctgtgtctgcactgtggcgggaacaggcacttcccacacttcctacaagtcctcccgctcccctgtccttagctgctgttcagctagaaaactgcttgatttatggctgttcgagacaaactgctaactcagcaatgggaatccattgccattcctcaggttcacacatgcttcctttcccaaggggacaagcttggcctaggaggtaattctagcattgccatgcctctgacttaaatcatagggcaagacaatgaaactatccaggtcatgttccccagctatagggaaggcaggtctaccctgttttgcacaagatgtgtgatcctgattaatttgatggttatttaacttttgcaaactaaatccttgtgtaaaggctgggaacttcctattttaaagaaatttgaaaagaaatttggcatggaaagatttattcccttcttaatctttcttcaagtactgatatgaaggtatggatgtgcttcagtaaattaaataccattaccagtgtttagtttagtggtcctgaccagcaatgctacttaatgaaacagaagaaaataccagaatgcatcatatgtaaaaagagtaagtattatttcataaaatttgtgtgtgtctgtgtgtacacatatgtatgagtgtttaagttatgacataaaacaaatttcttattgtgggtcacagtcaaagtttaaaagccactgatacatggtaatattatttaaatattttccggcatattaggtatatttaagatgtgagttccaaacaagatgctttattattttaagccaacgttttccaaacttttttgactgaggttcattgtaagaaacacatctttgttggtggaggggtgggacagggtctagctctgttgcccaggctggattgcagtggcgagatcatggcttactgcagcctcaaactcctaggctcaagcgatcctcccactagagcaccaggttgggaagagtgacagcaaccagggcctcagccctccaccccatcccccagtagctgagactacaggcttgtgcaagatgcttagctaatgttcgtattttttgtagagacagggttttgccatgttgcccagtctggtctcaacctcctcagttcaaatgatctgcctcctttggcccctcccaaagtgttgggattacaggcgtgagccaccgcgcccggccaagaaacacatttttaagttgtaatttcatactcacatgccacacacatacaactacacaacataaatga

SEQ ID NO: 19108 - RNA, 6888 nt, Homo sapiens
  source 1..6888: mol_type = other RNA
tggggcggggcaggtccctgcggagaggcacttctggcctgaagacagctccattgagcccctgcagtacaggcgtagtgccttggaccaagcccacagcctggtaaggggcgcctgccagggccacggccaggaggcattccccgaagccttgctcccctggtgcagcagggctgtgggaggtggtgacattgaggccagcctctttcaccagcagcttagcgttcaccaagttcacatccgcctgcttggaagcctctttcaggaggccgacaatgactgcggggcttaggcagttcccagcattcttcagggatgttccctgtgttatcacctggatggtccctttgggggacccagcccaggctcgcatcagtgtccccagagcttctgccagaccaatccaaggcttggtgtgtggagagaaggcactggtaagggcctgggcattcacaacccccgtgagagatttccccttcaccatgtccacgaactgaacagcaatttcctccccacagcggctctgagcctccttggtgctggcacccaggtggggacagctgatgacattctcatggtccaccaaggcccggtcccgtggcggctcttccgtaaacacgtccagtgcagccccggcacactggccagactgcagggcccggagcagggcgccttcgtccacgatccctccacgggcacagttcaccacacgcacccccttcttgcactgggcaaaggtgttgtcattcagcaagcctgtcgtggagggcaggagaggagtgtgcacagtgatgaaatcacagagaggccagatctcctccaggggcagctgctgaacaccaaaggaggccgagacctctggggaaatgatggggtcataccctatagtcttcatcccaaaggactgcatccgggtagctacctctctcccaatcctgcccaggccaagaattcccagggtctttccattcagctctgttcccatgaacttcttccgctcccatttgccgtccttcatcgaagccgtcgcctggggaatctgcctttgatgagtgaggtcatggtgagcagttgacaatggggagcttcttttaaaccacagcatttcaccgattcctttaaacaaagctggtccagagagctcagatggaaactgcagggaggagttagagcagaggtaaattcccccagatcctcctccagcaggagggaaagcaggtctcgccatgggaaaagtaatttcttggtcccggaaggtttcaggcctggccaggcacatgatcattccacaagtgagttctgcggcactgaggctgttcccattgggggtgttcataaccaagatgcccttccttgttgcggcctccagatccacattgtccacacctgtgccagccctgcccaccacctggagtttctcagctgcgttgatgacatcagcggtcaccttggtggcagagcgaacaataaggccttcacagtcctgtaaaataaaagagatggagcacatggctcctcagatccattttccccgtagagctctcagctggatcccatgaaaaccttcttttaccttcattcccactgcatggattctggagatagagaaaggtcatgagaagttggcttctagggtaagggcccacactgtgtttgttgtgcacgagcctagagcataggagcaaatatggacaaagtaaatgtaaggagagcagtgggtaattttatctccactaagaagagaagaggaatgatgcttaggctgcagcatagaatatttaagccttaagagcttctaaacactggaagaattgttcaagagcaatagtagaacgattcctctggaggtgtttatgcatcacacatcctcactgcttgggggctgtgcctaccagcagagagaaacatgcaggcggcctggaagacactccaaatccttttatgtctgaggttctgaagcagaacgtcagagtgggagatttgaagaaatgttcaccagcatctggtccaactccattttacagaggaaaaactgaagcccaacaaagttaagcctgcctactttcccttcccctcccctgtacttttcttccttcattttatcggatgcccgctatgtacgtatctggcattatgctaaactgattatgacctgggtgtatacaagtcacatgggcacccagggcttagaggaatcaaacagaagccacctcagtgctgactgccccagtgctgaggccaacaccaggtgagcacctggaggtattctgatttccccccatagcagcctagttaaatatcagccaagccaggcagaaacaggatactggcatcttttccacattcaagtccaccacacaggctccaaagaaaaggatttccctgcctggacacactttactgacttttcaaggtgcaataaagttatcttccaggaaacatttgccaacaaccctgaactgtcactctccctacaccccaccatttttgttgtgatcaccaatataatatgtttcatatctagttgtcctctcttagacctgcagttttggtctccttagttatattttctatgcctaatgcagggattttatattaaaactttatctactctataccatatatccatagtaccagcctcaccagcacataaaccatttattgagcacctgctgggtactaggcattacaccagttgctttacattattctcttcacaactccaaggagaaggggtataatcatccccagtttccagataaagaaacagaggctttgagaggtaacctgcccaaggtcactcttacagatcaaaaaccagccaagaactggaaagtcattgccactggctaactctgagactgtaactgaagaagagttggtagacctgccaagatgtcaagaagatagggccagagccaaggccatggccagttaggtgcaaaaaccaaactgtaaaatcccttggagagatttactagtaacaatagctaccattttttgagcaagtactttacatccagcactgtgcttcacaacaatcctaagacagatattacaattatccctatagtacagacaagcaaactgacacttaaagaatttagagaacttgctgaagtcacatagctaggatatggcagaagctggaatcaagtccaaatctgttgagttccaactaccttccaaatacagcatttagacacctaaaccaggagagacattgccagaaatcctgtggcttctccaagatggcagaagctccctaacaaaggtccctggatcttctggtgacctgctcctcccagccagcctgcctactgggggataatagaaataggcacaaatgcctctgtcgagaagagcaagttgcctgtggcctgtaggcaagctcacagttgatacttcacaatgaagtgttttatacacttccattgaataaatgaattcagtgatgagaggccggtagaaaccaccctcatcagtcccccatcctcacaccttcaccctctttcccaaataactttaacacttcacatgcctgaaaattgctcatcagaaatcccttcctttgactgtgataaggaggcataaggtctacttctaagagtgctcaaggattttcaaaaatcttattaaaagaagttgaaaaaaagcaggaaaaacgttcagaaattgacaaatcagtcaacagaactaaatagacactagacaaacagaatatgtgagaatttagaaaataaaaagcagaactcaaattgatgcggaaaggaagaactaaacaagaaataatgttatgaaaattcaagaagaaaaataatagattgctacctcacttcagatttttaaaaatccagatgaattaaagaatttttaaaaatataagcattaaaagaaaatgtcaggggatatttttatgactcggattgggaaaacctttcataagcaaggcacaaatcttagaaactctggaagaaaatattgacaaatccagttacattcaaattttaaacttctgcatggaaaaagatcccataaacaaaagcaagtagtggtcctgatatgtggagaaaactcctttcaccatatgtaacagaacaaggattcatcaccaaaagtgatagaattcctacaaatcaactttttttttttttttttttttttttttttgagacagagtttcactcttattgcccaggctggagtgcaatggcgcgatcttggctcactgcaacctccgcctcccgggttcaagcgattctcctgcttcagcctcccgagtagctgggattataggcatgcaccacaaatccacttttttaaaggataaagagcacaataaaaaatagataaatatataaataggcaatgcacagaagaactacaaagtggtcactagtttcactagtttatagactcttcaacgctagatatcaaggaaatatagatttttaaatatgatatttttgggcatcattttggcagaaagaaaatgaataatattcagcattggtgagcatggagggaaacaggagtgtacactgcatgacctttttggagggcaactgggcagtgggtgggtaagcacatttttagtggtcatttctttgcagccagcactgacaccttagaaaattggtaacacactgaggaaacacaacctcctttcaagtggtcagctcaggaccaaaagtcaaagttcaactgacaagaagcaggcatggagcaagaggagaagggaccacccagagtcatcatcttatcaccttgtctctctagcatcaagttccagagcccacatctcaggcccagtcctgctccagaggctctaccaatcactcccttgggccttaagggtccatccttcttcaatgttctctccaaagctgccaaaatgctccccaaaccttgcaaacctgctccccacaggcaacactagctggagagcatgcagactccccaaagtccacccattcttgtagcccctgaacaagcacagaaacagcactattgtttctttcatgagcatggactctctggatggatctcccttgtaaagatttatgctgtagtctcttcacttttccctcaaaccagccttctttggtgccagggaaactaagagtccccagtcagactcctacagatgagcatcaggtctcacctctcccaagggcagaaactgtcactcaggagaccttggtcccacattagaaccagacatcccacatcagtcagagttaatgagcttccaaggcctcttacaacctcaactacccactctatccactcattcaatcagcacatattcacagacagcctgaatccaacctacctcctgctggaccctcaaagcccctgcacccaagccccttccctcctcacgccacaacgcacccccttcaaagactttgccccaagctgtctgctcctgtcctctacttatggaaaccacagccctaaccaaatgcacccatctgctcacatcctctgcagtttgcgattaaaacttctccagtgtccagagatcctcccctctctttgtcattccttgggtgaggaagcaagtctctctctacacagcaccaaattctgatgttcactgccctctgcgtgtggcttctgtgtctgcactgtggcgggaacaggcacttcccacacttcctacaagtcctcccgctcccctgtccttagctgctgttcagctagaaaactgcttgatttatggctgttcgagacaaactgctaactcagcaatgggaatccattgccattcctcaggttcacacatgcttcctttcccaaggggacaagcttggcctaggaggtaattctagcattgccatgcctctgacttaaatcatagggcaagacaatgaaactatccaggtcatgttccccagctatagggaaggcaggtctaccctgttttgcacaagatgtgtgatcctgattaatttgatggttatttaacttttgcaaactaaatccttgtgtaaaggctgggaacttcctattttaaagaaatttgaaaagaaatttggcatggaaagatttattcccttcttaatctttcttcaagtactgatatgaaggtatggatgtgcttcagtaaattaaataccattaccagtgtttagtttagtggtcctgaccagcaatgctacttaatgaaacagaagaaaataccagaatgcatcatatgtaaaaagagtaagtattatttcataaaatttgtgtgtgtctgtgtgtacacatatgtatgagtgtttaagttatgacataaaacaaatttcttattgtgggtcacagtcaaagtttaaaagccactgatacatggtaatattatttaaatattttccggcatattaggtatatttaagatgtgagttccaaacaagatgctttattattttaagccaacgttttccaaacttttttgactgaggttcattgtaagaaacacatctttgttggtggaggggtgggacagggtctagctctgttgcccaggctggattgcagtggcgagatcatggcttactgcagcctcaaactcctaggctcaagcgatcctcccactagagcaccaggttgggaagagtgacagcaaccagggcctcagccctccaccccatcccccagtagctgagactacaggcttgtgcaagatgcttagctaatgttcgtattttttgtagagacagggttttgccatgttgcccagtctggtctcaacctcctcagttcaaatgatctgcctcctttggcccctcccaaagtgttgggattacaggcgtgagccaccgcgcccggccaagaaacacatttttaagttgtaatttcatactcacatgccacacacatacaactacacaacataaatga

SEQ ID NO: 19109 - RNA, 1612 nt, Homo sapiens
  source 1..1612: mol_type = other RNA
tggggcggggcaggtccctgcggagaggcacttctggcctgaagacagctccattgagcccctgcagtacaggcgtagtgccttggaccaagcccacagcctggtaaggggcgcctgccagggccacggccaggaggcattccccgaagccttgctcccctggtgcagcagggctgtgggaggtggtgacattgaggccagcctctttcaccagcagcttagcgttcaccaagttcacatccgcctgcttggaagcctctttcaggaggccgacaatgactgcggggcttaggcagttcccagcattcttcagggatgttccctgtgttatcacctggatggtccctttgggggacccagcccaggctcgcatcagtgtccccagagcttctgccagaccaatccaaggcttggtgtgtggagagaaggcactggtaagggcctgggcattcacaacccccgtgagagatttccccttcaccatgtccacgaactgaacagcaatttcctccccacagcggctctgagcctccttggtgctggcacccaggtggggacagctgatgacattctcatggtccaccaaggcccggtcccgtggcggctcttccgtaaacacgtccagtgcagccccggcacactggccagactgcagggcccggagcagggcgccttcgtccacgatccctccacgggcacagttcaccacacgcacccccttcttgcactgggcaaaggtgttgtcattcagcaagcctgtcgtggagggcaggagaggagtgtgcacagtgatgaaatcacagagaggccagatctcctccaggggcagctgctgaacaccaaaggaggccgagacctctggggaaatgatggggtcataccctatagtcttcatcccaaaggactgcatccgggtagctacctctctcccaatcctgcccaggccaagaattcccagggtctttccattcagctctgttcccatgaacttcttccgctcccatttgccgtccttcatcgaagccgtcgcctggggaatctgcctttgatgagtgaggtcatggtgagcagttgacaatggggagcttcttttaaaccacagcatttcaccgattcctttaaacaaagctggtccagagagctcagatggaaactgcagggaggagttagagcagaggtaaattcccccagatcctcctccagcaggagggaaagcaggtctcgccatgggaaaagtaatttcttggtcccggaaggtttcaggcctggccaggcacatgatcattccacaagtgagttctgcggcactgaggctgttcccattgggggtgttcataaccaagatgcccttccttgttgcggcctccagatccacattgtccacacctgtgccagccctgcccaccacctggagtttctcagctgcgttgatgacatcagcggtcaccttggtggcagagcgaacaataaggccttcacagtcctttcctccgaaggctcccaggaggcagaggggcggcgaaagcacggagcagtcttgcatcagacgaggggcgggtacgtgtttgctgccttacgagggctgccttcccctccagctgccccagcagcc

SEQ ID NO: 19110 - RNA, 1729 nt, Homo sapiens
  source 1..1729: mol_type = other RNA
tggggcggggcaggtccctgcggagaggcacttctggcctgaagacagctccattgagcccctgcagtacaggcgtagtgccttggaccaagcccacagcctggtaaggggcgcctgccagggccacggccaggaggcattccccgaagccttgctcccctggtgcagcagggctgtgggaggtggtgacattgaggccagcctctttcaccagcagcttagcgttcaccaagttcacatccgcctgcttggaagcctctttcaggaggccgacaatgactgcggggcttaggcagttcccagcattcttcagggatgttccctgtgttatcacctggatggtccctttgggggacccagcccaggctcgcatcagtgtccccagagcttctgccagaccaatccaaggcttggtgtgtggagagaaggcactggtaagggcctgggcattcacaacccccgtgagagatttccccttcaccatgtccacgaactgaacagcaatttcctccccacagcggctctgagcctccttggtgctggcacccaggtggggacagctgatgacattctcatggtccaccaaggcccggtcccgtggcggctcttccgtaaacacgtccagtgcagccccggcacactggccagactgcagggcccggagcagggcgccttcgtccacgatccctccacgggcacagttcaccacacgcacccccttcttgcactgggcaaaggtgttgtcattcagcaagcctgtcgtggagggcaggagaggagtgtgcacagtgatgaaatcacagagaggccagatctcctccaggggcagctgctgaacaccaaaggaggccgagacctctggggaaatgatggggtcataccctatagtcttcatcccaaaggactgcatccgggtagctacctctctcccaatcctgcccaggccaagaattcccagggtctttccattcagctctgttcccatgaacttcttccgctcccatttgccgtccttcatcgaagccgtcgcctggggaatctgcctttgatgagtgaggtcatggtgagcagttgacaatggggagcttcttttaaaccacagcatttcaccgattcctttaaacaaagctggtccagtgaatatcagtgaataccagagagctcagatggaaactgcagggaggagttagagcagaggtaaattcccccagatcctcctccagcaggagggaaagcaggtctcgccatgggaaaagtaatttcttggtcccggaaggtttcaggcctggccaggcacatgatcattccacaagtgagttctgcggcactgaggctgttcccattgggggtgttcataaccaagatgcccttccttgttgcggcctccagatccacattgtccacacctgtgccagccctgcccaccacctggagtttctcagctgcgttgatgacatcagcggtcaccttggtggcagagcgaacaataaggccttcacagtcctgcagctccgctatcagctcctctttgctaaggttctgcttttccaccacctgcagccctccatcttgcaagatcttccggcagcaagggtccaggctgtcactgatgagcactttccgcagatttgcaaaagccattgctggagttggcctcggaatcggccgctgtgagtagaagtacctaagccaagaagctgcggttcggcctggcgcgctagagtaactg

SEQ ID NO: 19111 - RNA, 1332 nt, Homo sapiens
  source 1..1332: mol_type = other RNA
tgggggagatgggggttgattcttctacagacatttgtatagttgtcatagtgtccccaggaatagagaggactgcgagattaggctcagaccccggttccaagactggggatggtgatggggtcggagaaggcgacgaaggctgggattctgaagggctatgctctgggccaggcagccctggccggtcagcaatgattgctccctgtgaccggtcatctggccggacaatgacagcaacctggggcgtctccccattagcttgaggctccagaccgcctcccgtctggggaggggtgggtgtggaggcagtgcgggccccagacatgatctcctctgtgatatcctttcctccttggtttggatctcgaattcggatcgtcttacgctccctcttgggagcaatctggggtggctggttcatcaaaactggggcgggggccacgccagtgggaaactgctgcaccccttgggctggatagtaggcgccagcgtaggtcccaaattctgtagggcttgcacctggatagaagcctggggctcctggctgcacagggtactgctgtgtcgggacaacgtatgtggaacgcccctgtccagggatgtagtaggccccctgggaggctgggtaggagatctgggaagggatcatcattacttgggatccagcagggtagacatgggcagctgggccagggcgggcaggggctgcactctgcactcgggaggctgcactgctcgggggctgggcccggctagggtagaagtgctggcggggctgagaaggcgtgttcatttgtgtcgcttgtggcgtactgaacaccaccggcgctgtctgccccgggggaaacgctggctgtgggagtccgggggatggggcgggtggggggcctgtggactgtggagctttgttcatttcatttggtgccacatcagggtccccccagcaccccctcgattaagaacaagtccacggtgcggcctacaggttctgggcatccgagggcctggggttgggaggtgagggtatcaacctggctccgcggggccccagaccaaccagaccggaaattccaggtctcgctggcaccaggctcccggatcacgaacggagctagctgcttcggccgtggcgtccccaccccccacccggggacaccgggttcgggcctggcccaggggcacacaggatacgcctgccgccggggaacccgcactgggccagaagctaggcctgccgccgcccaggagtgtaggccaggaagggcgggagtcaggccctaaaaggccaggcgggcggcggccgtcgaggagccggtttcaggcaagtga

SEQ ID NO: 19112 - RNA, 1097 nt, Homo sapiens
  source 1..1097: mol_type = other RNA
tgggggagatgggggttgattcttctacagacatttgtatagttgtcatagtgtccccaggaatagagaggactgcgagattaggctcagaccccggttccaagactggggatggtgatggggtcggagaaggcgacgaaggctgggattctgaagggctatgctctgggccaggcagccctggccggtcagcaatgattgctccctgtgaccggtcatctggccggacaatgacagcaacctggggcgtctccccattagcttgaggctccagaccgcctcccgtctggggaggggtgggtgtggaggcagtgcgggccccagacatgatctcctctgtgatatcctttcctccttggtttggatctcgaattcggatcgtcttacgctccctcttgggagcaatctggggtggctggttcatcaaaactggggtgggggccacgccagtgggaaactgctgcaccccttgggctggatagtaggcgccagcgtaggtcccaaattctgtagggcttgcacctggatagaagcctggggctcctggctgcacagggtactgctgtgtcgggacaacgtatgtggaacgcccctgtccagggatgtagtaggccccctgggaggctgggtaggagatctgggaagggatcatcattacttgggatccagcagggtagacatgggcagctgggccagggcgggcaggggctgcactctgcactcgggaggctgcactgctcgggggctgggcccggctagggtagaagtgctgcagagacctgaatcctccctggcggggctgagaaggcgtgttcatttgtgtcgcttgtggcgtactgaacaccaccggcgctgtctgccccgggggaaacgctggctgtgggagtccgggggatggggcgggtggggggcctgtggactgtggagctttgttcatttcatttggtgccacatcagggtccccccagcaccccctcgattaagaacaagtccacggtgcggcctacaggttctgggcatccgagggccttcagtctccttcagtccgcgcggccgagccccacgcagccgcacagacgtagtccacaaccatttcc

SEQ ID NO: 19113 - RNA, 1040 nt, Homo sapiens
  source 1..1040: mol_type = other RNA
tgggggagatgggggttgattcttctacagacatttgtatagttgtcatagtgtccccaggaatagagaggactgcgagattaggctcagaccccggttccaagactggggatggtgatggggtcggagaaggcgacgaaggctgggattctgaagggctatgctctgggccaggcagccctggccggtcagcaatgattgctccctgtgaccggtcatctggccggacaatgacagcaacctggggcgtctccccattagcttgaggctccagaccgcctcccgtctggggaggggtgggtgtggaggcagtgcgggccccagacatgatctcctctgtgatatcctttcctccttggtttggatctcgaattcggatcgtcttacgctccctcttgggagcaatctggggtggctggttcatcaaaactggggtgggggccacgccagtgggaaactgctgcaccccttgggctggatagtaggcgccagcgtaggtcccaaattctgtagggcttgcacctggatagaagcctggggctcctggctgcacagggtactgctgtgtcgggacaacgtatgtggaacgcccctgtccagggatgtagtaggccccctgggaggctgggtaggagatctgggaagggatcatcattacttgggatccagcagggtagacatgggcagctgggccagggcgggcaggggctgcactctgcactcgggaggctgcactgctcgggggctgggcccggctagggtagaagtgctgcagagacctgaatcctccctggcggggctgagaaggcgtgttcatttgtgtcgcttgtggcgtactgaacaccaccggcgctgtctgccccgggggaaacgctggctgtgggagtccgggggatggggcgggtggggggcctgtggactgtggagctttgttcatttcatttggtgccacatcagggtccccccagcaccttcagtctccttcagtccgcgcggccgagccccacgcagccgcacagacgtagtccacaaccatttcc

SEQ ID NO: 19114 - RNA, 1136 nt, Homo sapiens
  source 1..1136: mol_type = other RNA
tgggggagatgggggttgattcttctacagacatttgtatagttgtcatagtgtccccaggaatagagaggactgcgagattaggctcagaccccggttccaagactggggatggtgatggggtcggagaaggcgacgaaggctgggattctgaagggctatgctctgggccaggcagccctggccggtcagcaatgattgctccctgtgaccggtcatctggccggacaatgacagcaacctggggcgtctccccattagcttgaggctccagaccgcctcccgtctggggaggggtgggtgtggaggcagtgcgggccccagacatgatctcctctgtgatatcctttcctccttggtttggatctcgaattcggatcgtcttacgctccctcttgggagcaatctggggtggctggttcatcaaaactggggtgggggccacgccagtgggaaactgctgcaccccttgggctggatagtaggcgccagcgtaggtcccaaattctgtagggcttgcacctggatagaagcctggggctcctggctgcacagggtactgctgtgtcgggacaacgtatgtggaacgcccctgtccagggatgtagtaggccccctgggaggctgggtaggagatctgggaagggatcatcattacttgggatccagcagggtagacatgggcagctgggccagggcgggcaggggctgcactctgcactcgggaggctgcactgctcgggggctgggcccggctagggtagaagtgctggcggggctgagaaggcgtgttcatttgtgtcgcttgtggcgtactgaacaccaccggcgctgtctgccccgggggaaacgctggctgaagaggggagaccagagttcagcaagaggggaagcccaggtggggcagaaacccaagctgtgggagtccgggggatggggcgggtggggggcctgtggactgtggagctttgttcatttcatttggtgccacatcagggtccccccagcaccccctcgattaagaacaagtccacggtgcggcctacaggttctgggcatccgagggccttcagtctccttcagtccgcgcggccgagccccacgcagccgcacagacgtagtccacaaccatttcc

SEQ ID NO: 19115 - RNA, 1076 nt, Homo sapiens
  source 1..1076: mol_type = other RNA
tgggggagatgggggttgattcttctacagacatttgtatagttgtcatagtgtccccaggaatagagaggactgcgagattaggctcagaccccggttccaagactggggatggtgatggggtcggagaaggcgacgaaggctgggattctgaagggctatgctctgggccaggcagccctggccggtcagcaatgattgctccctgtgaccggtcatctggccggacaatgacagcaacctggggcgtctccccattagcttgaggctccagaccgcctcccgtctggggaggggtgggtgtggaggcagtgcgggccccagacatgatctcctctgtgatatcctttcctccttggtttggatctcgaattcggatcgtcttacgctccctcttgggagcaatctggggtggctggttcatcaaaactggggtgggggccacgccagtgggaaactgctgcaccccttgggctggatagtaggcgccagcgtaggtcccaaattctgtagggcttgcacctggatagaagcctggggctcctggctgcacagggtactgctgtgtcgggacaacgtatgtggaacgcccctgtccagggatgtagtaggccccctgggaggctgggtaggagatctgggaagggatcatcattacttgggatccagcagggtagacatgggcagctgggccagggcgggcaggggctgcactctgcactcgggaggctgcactgctcgggggctgggcccggctagggtagaagtgctggcggggctgagaaggcgtgttcatttgtgtcgcttgtggcgtactgaacaccaccggcgctgtctgccccgggggaaacgctggctgtgggagtccgggggatggggcgggtggggggcctgtggactgtggagctttgttcatttcatttggtgccacatcagggtccccccagcaccccctcgattaagaacaagtccacggtgcggcctacaggttctgggcatccgagggccttcagtctccttcagtccgcgcggccgagccccacgcagccgcacagacgtagtccacaaccatttcc

SEQ ID NO: 19116 - RNA, 838 nt, Homo sapiens
  source 1..838: mol_type = other RNA
tgggggagatgggggttgattcttctacagacatttgtatagttgtcatagtgtccccaggaatagagaggactgcgagattaggctcagaccccggttccaagactggggatggtgatggggtcggagaaggcgacgaaggctgggattctgaagggctatgctctgggccaggcagccctggccggtcagcaatgattgctccctgtgaccggtcatctggccggacaatgacagcaacctggggcgtctccccattagcttgaggctccagaccgcctcccgtctggggaggggtgggtgtggaggcagtgcgggccccagacatgatctcctctgtgatatcctttcctccttggtttggatctcgaattcggatcgtcttacgctccctcttgggagcaatctggggtggctggttcatcaaaactggggtgggggccacgccagtgggaaactgctgcaccccttgggctggatagtaggcgccagcgtaggtcccaaattctgtagggcttgcacctggatagaagcctggggctcctggctgcacagggtactgctgtgtcgggacaacgtatgtggaacgcccctgtccagggatgtagtaggccccctgggaggctgggtaggagatctgggaagggatcatcattacttgggatccagcagggtagacatgggcagctgggccagggcgggcaggggctgcactctgcactcgggaggctgcactgctcgggggctgggcccggctagggtagaagtgcttcagtctccttcagtccgcgcggccgagccccacgcagccgcacagacgtagtccacaaccatttcc

SEQ ID NO: 19117 - RNA, 661 nt, Homo sapiens
  source 1..661: mol_type = other RNA
tgggggagatgggggttgattcttctacagacatttgtatagttgtcatagtgtccccaggaatagagaggactgcgagattaggctcagaccccggttccaagactggggatggtgatggggtcggagaaggcgacgaaggctgggattctgaagggctatgctctgggccaggcagccctggccggtcagcaatgattgctccctgtgaccggtcatctggccggacaatgacagcaacctggggcgtctccccattagcttgaggctccagaccgcctcccgtctggggaggggtgggtgtggaggcagtgcgggccccagacatgatctcctctgtgatatcctttcctccttggtttggatctcgaattcggatcgtcttacgctccctcttgggagcaatctggggtggctggttcatcaaaactggggtgggggccacgccagtgggaaactgctgcaccccttgggctggatagtaggcgccagcgtaggtcccaaattctgtagggcttgcacctggatagaagcctggggctcctggctgcacagggtactgctgtgtcgggacaacgtatgtggaacgccccttcagtctccttcagtccgcgcggccgagccccacgcagccgcacagacgtagtccacaaccatttcc

SEQ ID NO: 19118 - RNA, 746 nt, Homo sapiens
  source 1..746: mol_type = other RNA
tgggggagatgggggttgattcttctacagacatttgtatagttgtcatagtgtccccaggaatagagaggactgcgagattaggctcagaccccggttccaagactggggatggtgatggggtcggagaaggcgacgaaggctgggattctgaagggctatgctctgggccaggcagccctggccggtcagcaatgattgctccctgtgaccggtcatctggccggacaatgacagcaacctggggcgtctccccattagcttgaggctccagaccgcctcccgtctggggaggggtgggtgtggaggcagtgcgggccccagacatgatctcctctgtgatatcctttcctccttggtttggatctcgaattcggatctggggaaagaaagctataagatgagtgggaagcaggaagagcccacctctccaccctgccccaatcttaagactctgggccaactccccaccccccagcgggaagcaggtaggtaggtgccagaaaccccttgagttccactttcagcccatctggctgctctcgtagtccctgccccagctcccacccttaagagacccttgatctcacagagcagccctgtacatcacaatgcccctccctccctcatccctaccccaccagcagtccccaagtcagtggctgcacaccctggggcccaggacccccatctagaacccaatcggctcacttgtggctagtgtgcctgatctctgggggcagggc

SEQ ID NO: 19119 - RNA, 7005 nt, Homo sapiens
  source 1..7005: mol_type = other RNA
tgggggagtgcagtgattgtggtctgtattccaaattttagggcctgattagacagaaacagaaacacaccatagcattgcctttttgactgggtcatagtttttcagcctctgcataccccatattaatattcaatagatattaggatttaatcattcaatttgataggaatttctgacaggatctgcctgactctgatacttttctcaccagaattgctgatgagagtctgtattactcccagttcacactgagccaatgattatgtttgttgacattaggtagaaatataccttgtcttcccaaaaactgatctcagctcaggaagccttgctcttaaccaataggctatatttattcctaaaactgcatttttctcactttgcttgaaacacttttaactcctccttgtccaccccctcaggttattgcaatttattctggactaagatgagaacctctctctttggaaagcctaccctgactccccaaagttgggcatgactattcccatggcacgacttgaactttatattatccaaatgaaaaaacaaaaccctctagtcccttaagagtagcttaaatctcaacattgatatttgaggttaatgttttaattaatcttgaaacattaatctagacagactgatttcacagtccctaaaacactgtgttcaactgtaagattttacaagcaattcttcctgtctgtaaagtagtaaaggattttggcctcctttttacctattaaaatactaaataaagtccagttttaaaattaatttctgatatattcatcatggtcaaaatatatccaatatttgattatttctgtcacctccactgttaacactatgttaacaccttatctcttttaggggtaactgcaatacctcctaattggaatccctgctttggctctagcctctactttgtcagttcttaacacagcattcagaataagcctgtttaaatttgttagatcacttaaaaccctccagtggctttttacttcacttagaataaaagacaaagcctttacaattacttacaaggccctattacctttaatttccctctgttttcctcctcccttacagtgctgcagtacattccaggtccattcctagcctcagaccctttgcacttgctctaccctctacacagaattctttttccatggagagctccatggctcacttgctccctcacttgttttagtgagataacatcctgggatctgagtatgtgcatatgagcttctaccatatgatgttacataaccctgttctttacaagccccctaatagtatgaaactctatttccatagaacatattcctgtagaattactgtagcaaagagtaacagcaattttaaggctcaggattggccaaattgtttttccaaaaagtcgttatcaatttaccctcaacataagcataagtatacatcactccatactcttgctgaaaatggctattgtcatttttgttaataaaagtgatactgctttgctttaatctgtttatgttcttcgtcaaaattttaaattaggtgtccatttaattaaaaagagtttgtactgtcacaatcatggcaaatatttctcctatttttgtctgacttatatgtttttcacccagtttaaaaatttttatgtggtcaaattgtgtattttttctgagtgtttaaaaatccctctagagaattttaaatattttatagtggaacctcctttaaaaaaacaaaatcaagtcatttttgcatatgaagagataaaatgtggctacacttgcagttcttttgcttctgaagatactagtcttcatgaaaccacatggaggtccatggaacacagcttgaaaacctgtattcaatcaatgttttattctgatataggtcatgaaatgaaagtcttttttattaaagagttaaataatgatctcagcacaatttactgaataatcctcctattcgcagatctttatcatgtgtgaactctataagcatatgcactgtatgttcaaatacacatatataatccatacactggtatatttctaagctatttagtgacttagaatcctaactttttttttcaaatatacaattaaattctccattattacaacttcatataccaatatacaatttattatatgttagggcaatatcattaatctttcttacaattatctttgctcttctccaatgtctattttccttaaaagactagaacatctttatctcaaattcattgggattttcatgagatctgaaacaaatatataaattaggaacattcccttaaggaaaattaagactcctctagtcaagtcctcttttatatttccccgttttttattattttcattctgcatttttgtaaattaaaaaccagattttttgacaattacatttcctgaatattccaagaatttagaaaactaatgattttgtatttttgcccaacttaatgagtttaaattagtgcacttttcacctttaaaaacatattgtaggtactcctttatgtttgtctaataaaccttcacctggtctcacatttaagcaatatcacattttcatctgttatagcacataattagaaatttttaacccagtgttttcaacattttaaaatgaagcattgaacgtgttttgatacatttggctttaatcatcttgatccgtttattttaatattttaggccaacttcttggggatttttttggtagtcattgctacagagactgaataatttttgcttttatcttctcccattttgaaaggtatatgcactttttttagttttattaagttgtaattttaggtttgtaaaaaaaaaaaaaaaaggcctttcttaaattgtcattcaaaaagaaaatgttattatgagtccctgctatttaagatcagaaatgtggcacttatggtctctctccagttgccggatgtagcaactaaaaacagaaatgaccagttaaatttgaatttcaaatgtatgaaattttagtgtaagtcccatgcaatatttgggacacccttatactaaaacaattattctttgcttatatgaaattcaaacttaactgggtgtcctgacaaccttactctcctacccagactcagcatttgtacactttacactcagcatttgtatatttttattgcacatttaattttttgaagttttggaaactatccagacaactgcatatctaattgatttcagtgcttatcactagtccttttataccatgatttccacattcacaaactctctttaaggcacatatacgctacactgttttcttgcttatcaaaaatatttgtttcctgcacatatgaaagacacttttgttataaaactggtgataataaacttttcaaatctcaaaattctgaacgtgctgctccattgccttctgagttactgttgcagagctctgtatccaccctccctttctggttttgcagataaccagaatttttctttctgcatgcttttaattgcttctttctaacctgtttctaaggttgctttaatactggttttgcctaaaacttagtgaccatatacttttaactcagagaaagtttcttaatgtctttgatcattgattctatgccaaatgttctttcaccttccttagagacacctttaattctcacactggacctccatcctctgatattcatatctgttctttcttagtttccatctcattatccttttcagatacatttaagatcagatcaagtttatctattaactatcaattattttatattcttcagtgttactttttattgcatttattttgatacagtatttcagagctccctgaagtccttctttgttgtatctatttctcttttcactttagatactcttctctacttgtatatttctactctatctttactgagttcagattctctgttatgccactaaggacaccaacatttctggaaatttcctctgaagcctgcagcagctaattttcagggcaataagtttccaggtctttaggatgatattcttttcttcagtattgcaattccctctaattttcctaaacatgtccacttttttttctcttggtattacttcagcatatttgtgtatcaataattaagactgtgtattccgactaactctattctgagataatggccaaactctctttttacataattagcttcagggttcatcgttgcacagagttctgagttcaatgctgtccttgcagatatttctctattaccactctgttctactgagattaaataaaattctactgcttggatctctaattccgaaccaatggagtatcttccatttctagcacttttgtccatacccttcacaccttagagaaaattctgtacttcttgttgtttggtatctgaacctattattaagcgtggaaaaccggaaagggaagggatgagtgcactgtagtcacctcaaagtgaagcacccctgcaacagaaggatggtccctgggttttctggttgacagagataacaactcagatacactgtctcagacacaatgtcatacaatgctttcctatcttttattaggtggcttttgtccataaacaattgaattctaccggccaaaactgagttttaagttctatgtgtttccatcttttctgttacttcctagggagtttttaggggagttaagagatgtcgtttaacagttggccaaccagtttcaattcaaaccaaaatttaagtaaatattttgaagacagtgaaaatacaaaattgaacacacaatttcatgcacattaaaatgcacagaaaaaaagactagaatgaaatagaatgaagagttttctccttaaatgtttaatatatttatgactgtattatatttatagtaggtaaagaaaaatacactataattttaaatatatagggttttttctaaagatctccttttgaagcaaataattcttagtgggagataggggaaactataaatgttgcttgggattacttgtgttatttataagatttccttaacagcaggatttatagggtttaaaggttaggtaaactttgattaaagctgttaactaaatgaacaatatttataagtttcctcttctatgattattgtgaagatgtgaattatgatcaaatcccttataatattcacggcatttgtaaggtttctctcctgcatggactctttgatgaattcgaagagctgagctatgactgaaacctttaccacacttagcacattgataaggcttctctcctgtatggaccctctgatgaatgtgaagattagaactgtgactaaaaccctttccacaatcatgacatttatagggcttttctcctgtatggactctctgatgaatgagaagatgtgaacgctgactgaatcccttgccacactcttcacatttgtagggtttctctccagtatgtactctttgatgagtgtgaagctttgaactcttactgaagcccttcccacattcaggacaagtatagggtttctcccctgtatggactctctgatgaatgcgaagatctgagctgtgactaaagtcctttccacagtcatcacatttataaggtttctctcctgtatgcactctctgatgaatttgaagatttgagcgctgggtaaagcctttaccacagtcttcacatttataagacttctctcctgtgtgtactaactgatgaattcgaagatttgagctctggctgaaacccttaccacactcatcacacttatatggtttttctcctgtgtggactctctgatgaacatgaagtactgaactccgattaaaactcttaccacactgattacatttaaaaggcttctctcctatgtgaagtctctggtgaatgtgaagtaatgaatttctactgaggtctttatcacactcaattttatagaatttctcttctgtgtggactctttgatgattgtgaagactagagatctggctgaagctcttaccacatgcattacagctataaggtacctcccctatgtgaactctctgatgaaagtgaactccggagctctgatgaaagttaccgtcaacttcatcacatccgtacagcttcttacctatgtggtttcttggatgtctatacaagtctgatctctgagagaagcatgctttacagatggagcattgacagaggttttctccaggttgatttctcttgtggaaaacacaccgtgagttccaataataaattcctttacatttattacatccacagtacttttcttccattgaatctctcagtaggtcttcttgacatatcaccccaacatactgtggaagggcttcctccactgggatataagaatgctgaactatgagcttctgttctttttccatggagaggtttttcctggatatgccaagacggtatctgcccccttgaaaaccatgtgaaccactcatgtagatttctctaccatagtcttgagtggtttttgtttctaaggactgccaaggcataaaatttttatattttaagttcctgagacttttgctttcaaaagtcagttcatagttcccataccctggtacttgtgtggagagtattaaccattcctgacactgggaacgatcttgctgtgtgaggtctttggaatctgtcccttgaacagtttccccatagttctgattctcatacatctgggcgccagcattccaccagccttgccagtaggaaaaattttcatattctaagtatctgaatttttcttcttgggatttgtagctctcattccagtttttgacatgacatttgtgtagttctcccacatgacctccctgtagagtcttttttgagaagaatccaggaatttccactcctcccatgtaaaaataatagtcacatcttcaaatgttactgccatctggtcaaagatcaggctgtaaaatgggggcatgagcctttgccaccccagtccttccttgctgatcaa

SEQ ID NO: 19120 - RNA, 7247 nt, Homo sapiens
  source 1..7247: mol_type = other RNA
tgggggagtgcagtgattgtggtctgtattccaaattttagggcctgattagacagaaacagaaacacaccatagcattgcctttttgactgggtcatagtttttcagcctctgcataccccatattaatattcaatagatattaggatttaatcattcaatttgataggaatttctgacaggatctgcctgactctgatacttttctcaccagaattgctgatgagagtctgtattactcccagttcacactgagccaatgattatgtttgttgacattaggtagaaatataccttgtcttcccaaaaactgatctcagctcaggaagccttgctcttaaccaataggctatatttattcctaaaactgcatttttctcactttgcttgaaacacttttaactcctccttgtccaccccctcaggttattgcaatttattctggactaagatgagaacctctctctttggaaagcctaccctgactccccaaagttgggcatgactattcccatggcacgacttgaactttatattatccaaatgaaaaaacaaaaccctctagtcccttaagagtagcttaaatctcaacattgatatttgaggttaatgttttaattaatcttgaaacattaatctagacagactgatttcacagtccctaaaacactgtgttcaactgtaagattttacaagcaattcttcctgtctgtaaagtagtaaaggattttggcctcctttttacctattaaaatactaaataaagtccagttttaaaattaatttctgatatattcatcatggtcaaaatatatccaatatttgattatttctgtcacctccactgttaacactatgttaacaccttatctcttttaggggtaactgcaatacctcctaattggaatccctgctttggctctagcctctactttgtcagttcttaacacagcattcagaataagcctgtttaaatttgttagatcacttaaaaccctccagtggctttttacttcacttagaataaaagacaaagcctttacaattacttacaaggccctattacctttaatttccctctgttttcctcctcccttacagtgctgcagtacattccaggtccattcctagcctcagaccctttgcacttgctctaccctctacacagaattctttttccatggagagctccatggctcacttgctccctcacttgttttagtgagataacatcctgggatctgagtatgtgcatatgagcttctaccatatgatgttacataaccctgttctttacaagccccctaatagtatgaaactctatttccatagaacatattcctgtagaattactgtagcaaagagtaacagcaattttaaggctcaggattggccaaattgtttttccaaaaagtcgttatcaatttaccctcaacataagcataagtatacatcactccatactcttgctgaaaatggctattgtcatttttgttaataaaagtgatactgctttgctttaatctgtttatgttcttcgtcaaaattttaaattaggtgtccatttaattaaaaagagtttgtactgtcacaatcatggcaaatatttctcctatttttgtctgacttatatgtttttcacccagtttaaaaatttttatgtggtcaaattgtgtattttttctgagtgtttaaaaatccctctagagaattttaaatattttatagtggaacctcctttaaaaaaacaaaatcaagtcatttttgcatatgaagagataaaatgtggctacacttgcagttcttttgcttctgaagatactagtcttcatgaaaccacatggaggtccatggaacacagcttgaaaacctgtattcaatcaatgttttattctgatataggtcatgaaatgaaagtcttttttattaaagagttaaataatgatctcagcacaatttactgaataatcctcctattcgcagatctttatcatgtgtgaactctataagcatatgcactgtatgttcaaatacacatatataatccatacactggtatatttctaagctatttagtgacttagaatcctaactttttttttcaaatatacaattaaattctccattattacaacttcatataccaatatacaatttattatatgttagggcaatatcattaatctttcttacaattatctttgctcttctccaatgtctattttccttaaaagactagaacatctttatctcaaattcattgggattttcatgagatctgaaacaaatatataaattaggaacattcccttaaggaaaattaagactcctctagtcaagtcctcttttatatttccccgttttttattattttcattctgcatttttgtaaattaaaaaccagattttttgacaattacatttcctgaatattccaagaatttagaaaactaatgattttgtatttttgcccaacttaatgagtttaaattagtgcacttttcacctttaaaaacatattgtaggtactcctttatgtttgtctaataaaccttcacctggtctcacatttaagcaatatcacattttcatctgttatagcacataattagaaatttttaacccagtgttttcaacattttaaaatgaagcattgaacgtgttttgatacatttggctttaatcatcttgatccgtttattttaatattttaggccaacttcttggggatttttttggtagtcattgctacagagactgaataatttttgcttttatcttctcccattttgaaaggtatatgcactttttttagttttattaagttgtaattttaggtttgtaaaaaaaaaaaaaaaaggcctttcttaaattgtcattcaaaaagaaaatgttattatgagtccctgctatttaagatcagaaatgtggcacttatggtctctctccagttgccggatgtagcaactaaaaacagaaatgaccagttaaatttgaatttcaaatgtatgaaattttagtgtaagtcccatgcaatatttgggacacccttatactaaaacaattattctttgcttatatgaaattcaaacttaactgggtgtcctgacaaccttactctcctacccagactcagcatttgtacactttacactcagcatttgtatatttttattgcacatttaattttttgaagttttggaaactatccagacaactgcatatctaattgatttcagtgcttatcactagtccttttataccatgatttccacattcacaaactctctttaaggcacatatacgctacactgttttcttgcttatcaaaaatatttgtttcctgcacatatgaaagacacttttgttataaaactggtgataataaacttttcaaatctcaaaattctgaacgtgctgctccattgccttctgagttactgttgcagagctctgtatccaccctccctttctggttttgcagataaccagaatttttctttctgcatgcttttaattgcttctttctaacctgtttctaaggttgctttaatactggttttgcctaaaacttagtgaccatatacttttaactcagagaaagtttcttaatgtctttgatcattgattctatgccaaatgttctttcaccttccttagagacacctttaattctcacactggacctccatcctctgatattcatatctgttctttcttagtttccatctcattatccttttcagatacatttaagatcagatcaagtttatctattaactatcaattattttatattcttcagtgttactttttattgcatttattttgatacagtatttcagagctccctgaagtccttctttgttgtatctatttctcttttcactttagatactcttctctacttgtatatttctactctatctttactgagttcagattctctgttatgccactaaggacaccaacatttctggaaatttcctctgaagcctgcagcagctaattttcagggcaataagtttccaggtctttaggatgatattcttttcttcagtattgcaattccctctaattttcctaaacatgtccacttttttttctcttggtattacttcagcatatttgtgtatcaataattaagactgtgtattccgactaactctattctgagataatggccaaactctctttttacataattagcttcagggttcatcgttgcacagagttctgagttcaatgctgtccttgcagatatttctctattaccactctgttctactgagattaaataaaattctactgcttggatctctaattccgaaccaatggagtatcttccatttctagcacttttgtccatacccttcacaccttagagaaaattctgtacttcttgttgtttggtatctgaacctattattaagcgtggaaaaccggaaagggaagggatgagtgcactgtagtcacctcaaagtgaagcacccctgcaacagaaggatggtccctgggttttctggttgacagagataacaactcagatacactgtctcagacacaatgtcatacaatgctttcctatcttttattaggtggcttttgtccataaacaattgaattctaccggccaaaactgagttttaagttctatgtgtttccatcttttctgttacttcctagggagtttttaggggagttaagagatgtcgtttaacagttggccaaccagtttcaattcaaaccaaaatttaagtaaatattttgaagacagtgaaaatacaaaattgaacacacaatttcatgcacattaaaatgcacagaaaaaaagactagaatgaaatagaatgaagagttttctccttaaatgtttaatatatttatgactgtattatatttatagtaggtaaagaaaaatacactataattttaaatatatagggttttttctaaagatctccttttgaagcaaataattcttagtgggagataggggaaactataaatgttgcttgggattacttgtgttatttataagatttccttaacagcaggatttatagggtttaaaggttaggtaaactttgattaaagctgttaactaaatgaacaatatttataagtttcctcttctatgattattgtgaagatgtgaattatgatcaaatcccttataatattcacggcatttgtaaggtttctctcctgcatggactctttgatgaattcgaagagctgagctatgactgaaacctttaccacacttagcacattgataaggcttctctcctgtatggaccctctgatgaatgtgaagattagaactgtgactaaaaccctttccacaatcatgacatttatagggcttttctcctgtatggactctctgatgaatgagaagatgtgaacgctgactgaatcccttgccacactcttcacatttgtagggtttctctccagtatgtactctttgatgagtgtgaagctttgaactcttactgaagcccttcccacattcaggacaagtatagggtttctcccctgtatggactctctgatgaatgcgaagatctgagctgtgactaaagtcctttccacagtcatcacatttataaggtttctctcctgtatgcactctctgatgaatttgaagatttgagcgctgggtaaagcctttaccacagtcttcacatttataagacttctctcctgtgtgtactaactgatgaattcgaagatttgagctctggctgaaacccttaccacactcatcacacttatatggtttttctcctgtgtggactctctgatgaacatgaagtactgaactccgattaaaactcttaccacactgattacatttaaaaggcttctctcctatgtgaagtctctggtgaatgtgaagtaatgaatttctactgaggtctttatcacactcaattttatagaatttctcttctgtgtggactctttgatgattgtgaagactagagatctggctgaagctcttaccacatgcattacagctataaggtacctcccctatgtgaactctctgatgaaagtgaactccggagctctgatgaaagttaccgtcaacttcatcacatccgtacagcttcttacctatgtggtttcttggatgtctatacaagtctgatctctgagagaagcatgctttacagatggagcattgacagaggttttctccaggttgatttctcttgtggaaaacacaccgtgagttccaataataaattcctttacatttattacatccacagtacttttcttccattgaatctctcagtaggtcttcttgacatatcaccccaacatactgtggaagggcttcctccactgggatataagaatgctgaactatgagcttctgttctttttccatggagaggtttttcctggatatgccaagacggtatctgcccccttgaaaaccatgtgaaccactcatgtagatttctctaccatagtcttgagtggtttttgtttctaaggactgccaaggcataaaatttttatattttaagttcctgagacttttgctttcaaaagtcagttcatagttcccataccctggtacttgtgtggagagtattaaccattcctgacactgggaacgatcttgctgtgtgaggtctttggaatctgtcccttgaacagtttccccatagttctgattctcatacatctgggcgccagcattccaccagccttgccagtaggaaaaattttcatattctaagtatctgaatttttcttcttgggatttgtagctctcattccagtttttgacatgacatttgtgtagttctcccacatgacctccctgtagagtcttttttgagaagaatccaggaatttccactcctcccatgtaaaaataatagtcacatcttcaaatgttactgccatctggtcaaagatcaggctttattaagtcttaacgtgggagagaagccgtgatgtacccatctacacgggtgtctctggggtttctaaaccggagtagcttctcagtccctgaccctcgattttctgcccctcttccttcaagcacagctcgtcttgccctgtccgcttctggctcagtcctcctgagagttcatgtcacttaacggagcctgtgagagtggaccgggatggccaaaacactcagtccacacaaacaatggccgcagcccggctggaccgaaacggaagtcccaggtcttggagtagacact

SEQ ID NO: 19121 - RNA, 7019 nt, Homo sapiens
  source 1..7019: mol_type = other RNA
tgggggagtgcagtgattgtggtctgtattccaaattttagggcctgattagacagaaacagaaacacaccatagcattgcctttttgactgggtcatagtttttcagcctctgcataccccatattaatattcaatagatattaggatttaatcattcaatttgataggaatttctgacaggatctgcctgactctgatacttttctcaccagaattgctgatgagagtctgtattactcccagttcacactgagccaatgattatgtttgttgacattaggtagaaatataccttgtcttcccaaaaactgatctcagctcaggaagccttgctcttaaccaataggctatatttattcctaaaactgcatttttctcactttgcttgaaacacttttaactcctccttgtccaccccctcaggttattgcaatttattctggactaagatgagaacctctctctttggaaagcctaccctgactccccaaagttgggcatgactattcccatggcacgacttgaactttatattatccaaatgaaaaaacaaaaccctctagtcccttaagagtagcttaaatctcaacattgatatttgaggttaatgttttaattaatcttgaaacattaatctagacagactgatttcacagtccctaaaacactgtgttcaactgtaagattttacaagcaattcttcctgtctgtaaagtagtaaaggattttggcctcctttttacctattaaaatactaaataaagtccagttttaaaattaatttctgatatattcatcatggtcaaaatatatccaatatttgattatttctgtcacctccactgttaacactatgttaacaccttatctcttttaggggtaactgcaatacctcctaattggaatccctgctttggctctagcctctactttgtcagttcttaacacagcattcagaataagcctgtttaaatttgttagatcacttaaaaccctccagtggctttttacttcacttagaataaaagacaaagcctttacaattacttacaaggccctattacctttaatttccctctgttttcctcctcccttacagtgctgcagtacattccaggtccattcctagcctcagaccctttgcacttgctctaccctctacacagaattctttttccatggagagctccatggctcacttgctccctcacttgttttagtgagataacatcctgggatctgagtatgtgcatatgagcttctaccatatgatgttacataaccctgttctttacaagccccctaatagtatgaaactctatttccatagaacatattcctgtagaattactgtagcaaagagtaacagcaattttaaggctcaggattggccaaattgtttttccaaaaagtcgttatcaatttaccctcaacataagcataagtatacatcactccatactcttgctgaaaatggctattgtcatttttgttaataaaagtgatactgctttgctttaatctgtttatgttcttcgtcaaaattttaaattaggtgtccatttaattaaaaagagtttgtactgtcacaatcatggcaaatatttctcctatttttgtctgacttatatgtttttcacccagtttaaaaatttttatgtggtcaaattgtgtattttttctgagtgtttaaaaatccctctagagaattttaaatattttatagtggaacctcctttaaaaaaacaaaatcaagtcatttttgcatatgaagagataaaatgtggctacacttgcagttcttttgcttctgaagatactagtcttcatgaaaccacatggaggtccatggaacacagcttgaaaacctgtattcaatcaatgttttattctgatataggtcatgaaatgaaagtcttttttattaaagagttaaataatgatctcagcacaatttactgaataatcctcctattcgcagatctttatcatgtgtgaactctataagcatatgcactgtatgttcaaatacacatatataatccatacactggtatatttctaagctatttagtgacttagaatcctaactttttttttcaaatatacaattaaattctccattattacaacttcatataccaatatacaatttattatatgttagggcaatatcattaatctttcttacaattatctttgctcttctccaatgtctattttccttaaaagactagaacatctttatctcaaattcattgggattttcatgagatctgaaacaaatatataaattaggaacattcccttaaggaaaattaagactcctctagtcaagtcctcttttatatttccccgttttttattattttcattctgcatttttgtaaattaaaaaccagattttttgacaattacatttcctgaatattccaagaatttagaaaactaatgattttgtatttttgcccaacttaatgagtttaaattagtgcacttttcacctttaaaaacatattgtaggtactcctttatgtttgtctaataaaccttcacctggtctcacatttaagcaatatcacattttcatctgttatagcacataattagaaatttttaacccagtgttttcaacattttaaaatgaagcattgaacgtgttttgatacatttggctttaatcatcttgatccgtttattttaatattttaggccaacttcttggggatttttttggtagtcattgctacagagactgaataatttttgcttttatcttctcccattttgaaaggtatatgcactttttttagttttattaagttgtaattttaggtttgtaaaaaaaaaaaaaaaaggcctttcttaaattgtcattcaaaaagaaaatgttattatgagtccctgctatttaagatcagaaatgtggcacttatggtctctctccagttgccggatgtagcaactaaaaacagaaatgaccagttaaatttgaatttcaaatgtatgaaattttagtgtaagtcccatgcaatatttgggacacccttatactaaaacaattattctttgcttatatgaaattcaaacttaactgggtgtcctgacaaccttactctcctacccagactcagcatttgtacactttacactcagcatttgtatatttttattgcacatttaattttttgaagttttggaaactatccagacaactgcatatctaattgatttcagtgcttatcactagtccttttataccatgatttccacattcacaaactctctttaaggcacatatacgctacactgttttcttgcttatcaaaaatatttgtttcctgcacatatgaaagacacttttgttataaaactggtgataataaacttttcaaatctcaaaattctgaacgtgctgctccattgccttctgagttactgttgcagagctctgtatccaccctccctttctggttttgcagataaccagaatttttctttctgcatgcttttaattgcttctttctaacctgtttctaaggttgctttaatactggttttgcctaaaacttagtgaccatatacttttaactcagagaaagtttcttaatgtctttgatcattgattctatgccaaatgttctttcaccttccttagagacacctttaattctcacactggacctccatcctctgatattcatatctgttctttcttagtttccatctcattatccttttcagatacatttaagatcagatcaagtttatctattaactatcaattattttatattcttcagtgttactttttattgcatttattttgatacagtatttcagagctccctgaagtccttctttgttgtatctatttctcttttcactttagatactcttctctacttgtatatttctactctatctttactgagttcagattctctgttatgccactaaggacaccaacatttctggaaatttcctctgaagcctgcagcagctaattttcagggcaataagtttccaggtctttaggatgatattcttttcttcagtattgcaattccctctaattttcctaaacatgtccacttttttttctcttggtattacttcagcatatttgtgtatcaataattaagactgtgtattccgactaactctattctgagataatggccaaactctctttttacataattagcttcagggttcatcgttgcacagagttctgagttcaatgctgtccttgcagatatttctctattaccactctgttctactgagattaaataaaattctactgcttggatctctaattccgaaccaatggagtatcttccatttctagcacttttgtccatacccttcacaccttagagaaaattctgtacttcttgttgtttggtatctgaacctattattaagcgtggaaaaccggaaagggaagggatgagtgcactgtagtcacctcaaagtgaagcacccctgcaacagaaggatggtccctgggttttctggttgacagagataacaactcagatacactgtctcagacacaatgtcatacaatgctttcctatcttttattaggtggcttttgtccataaacaattgaattctaccggccaaaactgagttttaagttctatgtgtttccatcttttctgttacttcctagggagtttttaggggagttaagagatgtcgtttaacagttggccaaccagtttcaattcaaaccaaaatttaagtaaatattttgaagacagtgaaaatacaaaattgaacacacaatttcatgcacattaaaatgcacagaaaaaaagactagaatgaaatagaatgaagagttttctccttaaatgtttaatatatttatgactgtattatatttatagtaggtaaagaaaaatacactataattttaaatatatagggttttttctaaagatctccttttgaagcaaataattcttagtgggagataggggaaactataaatgttgcttgggattacttgtgttatttataagatttccttaacagcaggatttatagggtttaaaggttaggtaaactttgattaaagctgttaactaaatgaacaatatttataagtttcctcttctatgattattgtgaagatgtgaattatgatcaaatcccttataatattcacggcatttgtaaggtttctctcctgcatggactctttgatgaattcgaagagctgagctatgactgaaacctttaccacacttagcacattgataaggcttctctcctgtatggaccctctgatgaatgtgaagattagaactgtgactaaaaccctttccacaatcatgacatttatagggcttttctcctgtatggactctctgatgaatgagaagatgtgaacgctgactgaatcccttgccacactcttcacatttgtagggtttctctccagtatgtactctttgatgagtgtgaagctttgaactcttactgaagcccttcccacattcaggacaagtatagggtttctcccctgtatggactctctgatgaatgcgaagatctgagctgtgactaaagtcctttccacagtcatcacatttataaggtttctctcctgtatgcactctctgatgaatttgaagatttgagcgctgggtaaagcctttaccacagtcttcacatttataagacttctctcctgtgtgtactaactgatgaattcgaagatttgagctctggctgaaacccttaccacactcatcacacttatatggtttttctcctgtgtggactctctgatgaacatgaagtactgaactccgattaaaactcttaccacactgattacatttaaaaggcttctctcctatgtgaagtctctggtgaatgtgaagtaatgaatttctactgaggtctttatcacactcaattttatagaatttctcttctgtgtggactctttgatgattgtgaagactagagatctggctgaagctcttaccacatgcattacagctataaggtacctcccctatgtgaactctctgatgaaagtgaactccggagctctgatgaaagttaccgtcaacttcatcacatccgtacagcttcttacctatgtggtttcttggatgtctatacaagtctgatctctgagagaagcatgctttacagatggagcattgacagaggttttctccaggttgatttctcttgtggaaaacacaccgtgagttccaataataaattcctttacatttattacatccacagtacttttcttccattgaatctctcagtaggtcttcttgacatatcaccccaacatactgtggaagggcttcctccactgggatataagaatgctgaactatgagcttctgttctttttccatggagaggtttttcctggatatgccaagacggtatctgcccccttgaaaaccatgtgaaccactcatgtagatttctctaccatagtcttgagtggtttttgtttctaaggactgccaaggcataaaatttttatattttaagttcctgagacttttgctttcaaaagtcagttcatagttcccataccctggtacttgtgtggagagtattaaccattcctgacactgggaacgatcttgctgtgtgaggtctttggaatctgtcccttgaacagtttccccatagttctgattctcatacatctgggcgccagcattccaccagccttgccagtaggaaaaattttcatattctaagtatctgaatttttcttcttgggatttgtagctctcattccagtttttgacatgacatttgtgtagttctcccacatgacctccctgtagagtcttttttgagaagaatccaggaatttccactcctcccatgtaaaaataatagtcacatcttcaaatgttactgccatctggtcaaagatcaggctttctgtaaaatgggggcatgagcctttgccaccccagtccttccttgctgatcaaaggtaggttc

SEQ ID NO: 19122 - RNA, 10697 nt, Homo sapiens
  source 1..10697: mol_type = other RNA
tgggggctgggatgggccatggttttggtggcaagatggacgctagaaatgtaggtttgtagttgtccacttagagaggggctttggactctgaggaagagggtgaagagagaggaagtccctggaacttaaattgagcctgtatttgagatggaggaaatccagagaaagaggccagtgatggcagaggagactcagatctgagtggtgtacaagccagaagaaagtacatttcaggaagaaaaagcctcagcatgcaaacagaaaaatagggttctttttcagttgtgatgtgcacgctgccttcttaaacggatgagattggacttcccttgggctgccttggagacctagtgctgtcattgtggattctggctgcgtgccgctgcctgaccccggaagggtgggctgtttcctccacctcaaggggtcctgactgctgggcttttgtgagcggcacattcttcctgccatcagtgtgtcaacctccagagctctgctgactccagttaatgtgctgcttctgacatgctgccaactggaagtcagtatttgggaaagagagaataaactatgtctaagaatgaaaagatagagattctcttgtggaaccctcaggggactcagtgacatgatgttgctactctggacccttctttgtgtcctctgtaccagggaggactccagataggtcatacatgctcatgaagacgttgctctgctggtctcacatggtcggaaggacttgagtgaagtggtcagcaaggaaacttaggtagacatggaaaatgggctgcctgtgggaagctcgcaggtcttttggagggaggtggcatttaatttgttaacaggattcatgcataatggtttagctgaaaccttcttcaagttcccttaaagccttggtcatctctgttgtttttctcccaaagaaatctctgccagtacatttttctttatgacatgcttattcatgtgaagaagtatgagtggttttctaatctgctttttctttgtagaaccaccaccacctaaaatccccaaaattgagaccactcatccaccgttgcctccagcccacccacctccaggtaagcatctgctgaagcagcttggccagctgtgcacatcgcctctgaatgttggacgcagcaggtcctgggaacttagaaaagggagactggggcccagattgacaatgtcagccacaggcaggaatctttgcaaaattgttcttgggctgggcacaatggcttgtgtttttgatcccagcactttgggaggcggaggcaggagaatcacctgaccccaggagttcgaggtcagcctgggcaacaaagtgagaccctgtctaaaaaattagccaggtgtggtagcacacacctgtagtcccaactacttaggagtctgagatgggaagatcatttgagccctgggcagtcaaggctgcagtgagctatgattgcaccaccgtactccagcctgggtgagagggagaccgtgtctcaaagttctgattttgaccaggtattttgagaatgttgtaaattgttaagtatatctgaatattttccgacctctcacatccagaaatgctaaactacacattgtattagaatcagttttaggaaagaaagccaaaccccgccttctgagatagaggcagggttactgtggctactaggctccggccgcccctacacctgcttcctattggcagtgtgtcgtcttagtgcattctgaagaataagcaattgtacagagagtaaatgaaagagtgaaaagttctcaacaagtagtacatggtaagctggaaagcctctctgataccgctggcaatagaggagaaaagctgtaaagtagatggcattctttacctgtggcaccatttcagaaggtgatgcgctagagaaggccagagtgacctgtgcttgctctccaaaaggtggtcgatactccggaggcttccaagcctctgtcagcagctcctccagcctgctacactcactgttggtcggtgcacgtggctcacactggggctgacagcactgtgtgcccgtaacagatgtgccacagattacatttctgttcctactcaatcatgatagtgtttgtgctttgggagaacagaggcgtcattttccactttggggccaaatcccaaaacccccaattcaatatgaaccttacttaaatgcctgtggttgctcatgaagcatttatggagcacctcctcgccaagtgcagttcccctggtccgagcctggggctgtgccttcactgaggagatgggtggtttatctggggagcctggggcagccacaggggtgctgctacctccagggcactgagtagctgctgtggaggcctcagagctctgctccctcccccattacagatagccaggagtaggcctgggacttgagtgggacctgggtgccagatacactgccaggaggccatggctgaagagagcagggcctgggaggcgcagtaaagctgggccgtgaggaagggagggaagtacgcttcctgggaggccctaggccatgggaagaggcattcaggtcagcagtgatgtttagggagcagtttggtggcagtgtgtgggacttggtcaggagcaagtgtacagagagggaatggggtgcccaggagagacccccacttgctgttccagctcagtcacacagcacaagggcaggcacactggtgacttgaagattcaggctacagggtcgagtgttggaaaagttgatttctgcaaggtggaggagcaggcctgtgggcccaggtggctgtggagtgacacacaggaggcattgaagggtgtcagcacttttctgcacctcttttttagtcagctcctagaaccacagggcatctggccctgacctggagccaaagccagttatctaaggccaggcacatatgaccttcctacccggtaggctggcggggtgctgatgtggcacaccagtggcacacctgttaccgacctgatgaaatcctgctcatgctcgctttggcaagatcaaacgggttgtgtgccaatggccacgtctacccaaccaggatgtcgtgctgtgccttgcctaacccaagtgcctggggaaccagaagcatcttcgtggctttgtcctctctatgttctctggaaccagaaatgttgctcctgtggtctgtctcctgggctgccttgggaaaggacactcattctgtgtgtttggctacctgtggtggggtgttgcgatgtcattttccagtggtctgacggtgacccgggatcacaggccaaaacatgttaaataaggctttggcagaagggggcgtgagggctcatgggttgggaggcgctgtgggaggggcctgaggctggttctgagcacgagtatcttgggcgtgctcaacacctagtgctgcctgtccctgctgcacacgcagcacgcacacacacgcagcacgcacagacatgcagcacgcacgcagcacgcacacgcacacacatgcacacactcctctcaaggaggctgctatctgagagcacacagtggggtttgatgtagcctctcttgagtagaatagaacctgaattgctgcttcgatgggtacaccgggaatgtcagagacttgtacagaattgttttaagtgccatcacattcatttgactaactctgaggttttctgcaaaatgccactgctgcagacaggagttcagtgtggccctgacccctggggtcagtttctgaaggcagaaaaacagaggagcccccacacgttttgcactaggaagagggggctggggccagggcacaagggggcttcgggtgctgccgagactgcctgtaggtggtgtggtcagggctgagggagggaaaaccccaggtcgtcgcagacagggtggagggccttcttgacagatggtggggagacatctggtggcatcaggacatggggcatgggcccatgcgttgggccacagaggaggcgggcagctgctccctgctcctctgtaaagatggccctgaagggccaggaggcactgaaaaagcaaccattgctggcggaggccgggcactgatgcgtctctctcctgcagaccggaagcctcccctcgctgctgccttaggtgaggctgagccgccgggccctgtggatgccactgacctccccaaagtccagattccccctccggcccacccggcccctgtgcaccagccaccgccgctgccacaccggcccccgcccccacccccctccagctacatgaccgggatgtccaccaccagctcctacatgtctggagagggctaccagagcctgcagtccatgatgaagaccgagggaccctcctacggtgccctgccccccgcctacggcccacctgcacacctgccctaccacccccatgtctacccgcccaacccgcccccgccacctgtgcctcctcccccagcctccttccccccacctgccatcccaccccctactcctggctaccccccacccccacccacctacaaccccaacttcccacccccacccccacgcctcccgcctacccacgcagtcccccctcatcctcctccagggttgggcctgccgccagccagctacccacctcctgccgtcccccctggaggacagcctcctgtgcccccgcccattcccccacccggcatgcctccagttggggggctggggcgggcagcctggatgagataacgtgagccttttttccctctttgtttttttaacaagattttctaatcgacttgcagagtagttgaagtgggtaagcagcagggtaccttgtataatgcacgacagttgcagtatgggaagaatggaccgggcccctgggataaaatcagagtggtcctcacacctagaggacggggacaaccagctttcagagtagcctcatcagtgcccttgcagtctgactgtgtacacttggttcagctaatgtctgagagtcctgcactgggttactttatactagtgaggacgttaaccagccatattggctcaataaatagcttcggtaaggagttaatttccttctagaaatcagtgcctatttttcctggaaactcaattttaaatagtccaattccatctgaagccaagctgttgtcattttcattcggtgacattctctcccatgacacccagaaggggcagaagaaccacatttttcatttatagatgtttgcatcctttgtattaaaattattttgaaggggttgcctcattggatggctttttttttttcctccagggagaaggggagaaatgtacttggaaattaatgtatgtttacatctctttgcaaattcctgtacatagagatatattttttaagtgtgaatgtaacaacatactgtgaattccatcttggttacaaatgagactccttcagtcagttatccaaataaaagcagttctgaaactatccctttctttgttatgggtggaaggtggggctccaggccttcgcagtctgtggcttataaaatgtgcagaggccctccttccagaccctggggacgcgggagaggcctggctgcagctcacagcagccacagccaaccccactgcctcccaaggcactctgggtggatccgcacagctgcctgccaagccagcctgcccccatcctgtgcctgccttggtttcctttggaggacctggttgagttccaaaccagtttgaaactttgaagccttgctgcgtagaacgcacacaggaacccgggggcttggatttgaaaccctttccacttctggcctgtgatgagacagaggcagctggaggagcagcggcctcactgtccaccttgaggggccacggctctgtctgtggaaggggccccgactgagcccccatctgcggtgcttgaggggccttggccctgtctctgcctgctgaccctgccacccacgacagaaacaagcactgagcacccagccaggaggctcacaaagaggcctttatttatctagctcaaagtagacactatcacaatcttgtttgttactccttttactaaaatagttcaaatcaatgtttttaccacactatcaaaaagttctatttcttcttgtctccccacgtcagagtggttgaatagaaggtagaaacaggccgggagtccacgggctcccagctctaaacggcgccagggcaggaaggggtggctccaggtctcactgtggcaccttctacagaaaatagacgtagctgccgggcccggggacagaaaccagacgttccagtccatctccaaaaagcagcacaaatactttgccccacagtatgaaaaatatacacctctaccgctctgcagtcatgcatttagttttaagaaaaaaaaaaaatcagtagtatgtatcttgtttcctcaagtttcaagaaaaaaaaaatgaaaggtcacttttttctctttaaacactgatgtgtagctagtaacttggataaaaaggtgccaccctacaaaatgtgctcagcatgttctgaggccaggatgggcttggccacctgggctggggcgaaaggagacctccatctgtcacagtggaaactgaagccgagtgccagtgccgcgtccggcttcaagatcaagagtcagagcctttgaaatggaaagggggcatctgaaagggcacccccactgggggctttcagagctaaggctccagaaggaagggggtcgccctgctagtgacggagctgggagtcaccctgagctacagcatgcccagatttcccctgtgggaagccccatctgaccttctacagcccacggctctgcaactgccacctgtactcaggtacatggcgtcgctgctgctggcttttaaaatcagctattagtttgagatgtgacagtcgccgacagggttctgtcctagaaagccatcccagtgccgtgttggctcaggggtcaccagctttgtgctgcctccgtaacagcaggagggttctcaaagcaatgttccactgatccctggatgccactgcagcattaaagacagggtcagtccccttgaggggaaaggtggcttcaaggctgttctctgggcctgtttgcaggagatccgcaggtaccaggagcccgtacttattgcttatttcagtggtggccacgccaacctgacccaaacatgatgcacacgggctcccagacttggctgccactcaaaatggacccacagcccttgggctactctgcggttctttggactgcaagacccagaggggcctctgctcagctgcccactcgggcaagaatcactgggtaccatgagcagcaggtgttcacccaacttcacgtgtacacccctagtgaccgggagcgcaccacctgaccgggcgacactccttcccaaagagcctcctggcaacacccacggcaggagcgccacaccatcccatcaccagcacccacttacccccctggggctaagatggggggcgtgagcctttcccctgagagcaaacgggcagcaagaactgctcagaatagagccgccagctagggagagggacagggcggccatctccctcctcttgcctgcatccccagccctgggcctgcatgagacctgctgggtaggaagacagcctctctgggctcttcaggtggggctgagcagcccctggaagagcacaggagtctgacgaggacctggtgaggtcctggacccaagagctagggctgcttacagtggcatgagcggatgtggggaagcggcctgtccccgtgctgcagctgtgggatcaaaatccctgtcatgtgccacacatcaccccctctaggccttactttcctcacacacacagttttctattgcactttacagtttatacatggtcatttacactgaagatctcacttgatgccagaatcctgtgaggagggccttatgctgcccattttactactgaggacacgggctcagagtggggaggcaactctccacccgcagcgactgcaaggcagcagaactcagctccacccggcccgccctcagccgtcggctgttggctcacgccccctcagtgaggacccctgccctgtggcgctggatgacctggagccataagcatggccgaaaaggaacctcagagacctgtttccaccaagagcccagacaggctgagtgaactgctaaaggtcacaccacaaactaaaggcagaacctggccagacacgctccttcccaaaaagaacagaactctcatctgcagcctacacagctctgtccacagggacccaagatgcagccaggccctgggggaggtcacagccaaccagagccccagctgtggcccagtgctgcccatcaggaaaatcacatgtggctcagcccagaaactctccccaggcccttcctgttactggcctgtcatgtaaaccacgaaaagggacgtgcctcaggcatggggcaggaggagcccaagaagggcatagcctggacagggtggcagggggacattgcagagactgggggggagggggatgacctccaaaagcaaggagcagcgggcatcgggtggctgagcacagatccccaggtgtgagggcaccctgacctccaaggctgagggtcacaggaagggcccagggcagcctccagccagccacagatgtggtgagtggccttgtccacatgccggggacccagtgcttggggggcctggggccaggccacggcatttgggcaagaagtggtgccacctgcgtcaagacccaggtagtggtggtctctgtccagtgtgggtggcagccggggagtagagggtttgatgagtggcccctccatcccaggcaggacagaggagcctggacagttcccaggctggatctcagaagcagcctgcagcctcttgctcatggagcccagggcccagagggggaatgaggcgtccgggccgctctgctgcaggaacagtcgcagcgtctcgtcttcccaggttgctggtgtatgaggcgggagatggcggcttgggccagtgcatcggacccatggcagctgggccagggcgggcagcgtcctatgtacagttcaccacagaggaagaagacaggggctgggctggaggtcctgcccgtgtctggggcctgaaactccccctggggacccccagcagggccagtccacgtccacagaagagtggccctacaaaggccccttgaactggttcccagacaggtgctgccgtatggagggcttggagctggctgcatctcccagctttctccagaccacgttgcacatctcgcgaacgatggccttctccttctcactcaggtcctcctcacagctgtcctggagctgccggtccagattctcgtgtacctccaggaccttcatggcatgcacgacagcctcgggcttctgtcctgcagggctgtagccagcagaggggggcgagggcagctcaggtgcggggcaggccgggccgttctgcagggagtcctggtaggagggcggcagggacgcaagctgggactccgagtggtagggcgagaagcctttccgcagcgtgcggaactctccggagcctgcctgctgtgcgaggagcttgtcaccctccagcagcctcactttgctctccagttgcctgatgtaggtggatgagggatcgtgcaggccgttggggatgctgcggtggtgcggcggcgccgacaagtcgtccagggaccgacgtgtggctcctgccttgccgtcgggggccttgtgcggcccggggggcagcagcgggggtgggacgtggtggtggtggtcggggctgccgccgctgcccgcgctggacgtactgctgccgtcgcccacgtcgcgggcccccgcgccgggcgcgccacccgacagcggcccgctcaggctggcctggctgtcgatggagctgcgggagccggcgccgcccccgccgccgccgccaccgcttgcggcccccgtcgccgccagtgccgcgcgctcctcgtccagcagcagcaccagctccttgagctccaggttctcgcgcagcagggcctcctggcgcgcctcgagctcgcgcagcttctgctgcgagcgggccacctcgtgccacacggcgccggccgcgtggcgcccgaagcgctgccactcgcgcgccagcttgcgccccttctgccggtcgtcgtcgaggaagcagcagagctcgcgcagctcctggttgtcgtcctgcagccgctggttcacgtccttgaggccgcggatctccagcaggtgctgctgcagccgccggttcacgtcgcgcatcaggccgccgtgctccagcatgaggcccaccttctcgccctcggcgcgccgcagccgccgcgccagctcctccttgctccagcgcagcagctcctcgtccggcacctggctcagctcctccgacgccgccgccgccgtcgccgcgggcttagccatggcggggccgtcaccgcggcatcgccctcgccctcgcccggccggcgcttccccgcgccggggctccgctgggccggtccgcgcgcgggcggggggcggccgggggcgcgtgcggcccgccccgcgccgcctggcgcgtcctctcgccgcgcccgccggggccgcccgggagcccgcgcgcctcggggttgacgagcggaggcggctgctgcgtcggcggccgcggtgccgggcgctctcagggttct

SEQ ID NO: 19123 - RNA, 50 nt, Homo sapiens
  source 1..50: mol_type = other RNA
tgggtggaagaaggtctggtttttcaggccttggagaagtatctgtagag

SEQ ID NO: 19124 - RNA, 2450 nt, Homo sapiens
  source 1..2450: mol_type = other RNA
tgggtgtaggctggagctgaggagccggcggcgggaggagccgggcaggctgccgtggcctggggatcctgagtcccgggagtgctgcctggccagggcctcggggaattccgccaggtacctcatgaaggagcggcccagtccctggcatgagctgcctcgcttcttgggcaggtgggggttgtttgcggccatttccttggttttgtggacctctagctgggcatagagcttcttcagctcgtcccgaatgtctccagggtccaggctgtgctcactccaggctgaggcgatgctgctgccaaggtaggagcctgagtgctgcaggtccagctcgtcctcacacacctcatccaccatctcctcccggggaggagcccccagcttccagaacttagggatgaagatcagagccagcgtggtggtgactgtgctgtgggtgtggaagaagaagaggaggagggtccagtccgggtgcagagagggaaccagcacaaacctggctgtgtggaaggcagcggaaagcagtagctcattgtgcagggcgatgcccatgtagcgtggctcatggaaggccgagagcacagcccgtgtggcgtagcagaggaagctgccccagcacagcagcagcagctcagccacaaccatgatgtagtcccagcggtcgtggtgacagaggtagaaatggcggccactgggagtgtggcctcggatcaccagaggtgcgtgctggatgcctcgctccagggcgcccacggtccacacagccaggaagcccagcacaggtagcaggagcagccccaggtgccgcagcagccgcccgctgctcagaagggcactccgctgggccgttcgagacagaaacagctgcagcactctgtaaagcttgagtatgatggtgccgtagacgatggcaaaacccagcagccgcacccagcgaagagcgatgcagcggaatacactgggcttgaagtataggatgaagacaggaaagtaaagcagcaggaatccaaaaaggacagtttccagcaggaccactccagatgcccagatcctcttgttccggcggcagcggtaggagaccagcatgctcaggaagatggccagcatgcagcaggcctggcaggccagcacagcggcccgcagcaccgcggcctcttccaccaggcacggtgtggcatccatgcagctggtgcagccctcaggacatggcagacactgcagcagtctcccagatctgccttctgggaacccgaattgcccggtagtctggaagtcactctcctctaaccccccagaggggcttgccccgtagaatccaggtcggcagcggcagaggtagcggccaagaacaaagccctgactctccagggggacacactgggtgctgttgagatcacacaggtgtgtgttagagtaccagcctgggccacttgcacactgattgatgtccacactctggagatctacgtccatctgcacctgccccctgacttctgggctgaggtctggcttgagtccatagaaggtggcagagagtgtgatcagccatccaggtcggagccgtccctcctggcattccaggaaaggaggagacagcctcacctgctgcgtgtcccccacatatccatctgcctgcggccacttggggctgccgaggctccctaggtcattggtcaacactcgcttcttcagggcaggggtgtccaggtccccaggagggttctcctcctgcacccagttcccagacaagtcctgcaggatggtttcctccccagtccgggtggcctgcagggccagctgtaggtggctggcccctggtggagggttaaaggtcagcaaagccctgtacactcttgggtccccctcggccacgctgcggaccagtgcctggtaccattccacatcctcctccacactggactcacggatgtcgttggcttgcagcagcatgttgagaaaattggcggcctgggcaagggtgcccgctgccccctgtaggcttggggggagccctggcatggctcctgccccacgcgcttcatagcgctcactgcaattcacctgtgatagctgctgggcatctccagagtagagataagcgagggcggcctcggccccctctaggggcacctgcatgggtacagatcctggcttgacttgggaagacagagggggcagagagcggatgggccgtggaccccccagagcccaggcacagacaaaacagcagcccagcagcccccacataggagggggcatgaccgctcccctggtgcccatccttggggcagctctcaggaccctggggtccaggctcaggagagcccaggcagaggctggctgcagtctgggggctgtcggcctccacgcctcctatgctggcgttccttcttcctctctccgtctccctctcacgctggtgccagctcgcctgcttttttcttctc

SEQ ID NO: 19125 - RNA, 398 nt, Homo sapiens
  source 1..398: mol_type = other RNA
tgggtgtaggctggagctgagggatctttcccctccaggcccttctgagaggtcctgctgtgtgcctcctgtcgtggcctcacatggggactccagtcccaagttaattctgggtgttgagcaacttggtctgccagcagccagggtccaggcagttggagaggtctcagctgaaggcccgtgttctgaagcacccaggacctccctaaaagcgtccctgttgcttccgatttcagatgggcttctttgaatcactttctcagcttccctgccttttgactacagttttcagctgtttgccttgtgttctatcatagccttgcctcagctctggaactcatttcaaattagatctaccacatgttgacgcttggcaaaggagccatttcactaaccca

SEQ ID NO: 19126 - RNA, 189 nt, Homo sapiens
  source 1..189: mol_type = other RNA
tgggtgtaggctggagctgagggcctagagtgagagggggcaaggcaagggggggagaggaagagaggcaggattagagagaggaggcaggccagaaagaggagagcaggagagacccaaagagaaacagaaggcagatagagagggagtgagaggcaggagctgagacacagatcctggaggaagaag

SEQ ID NO: 19127 - RNA, 2025 nt, Homo sapiens
  source 1..2025: mol_type = other RNA
tgggttcctggcatgctgatttttacaatgccaaacatccctctcgggaattaaaaatatttcaatctagtttagtcctttcgtactcttcttttgcgtactgactttatcggcccatctccagatcctgtgctctcatctgcttctttcatctcatcctctgacccagacttatttgattgattactttcttcttgcccttctatgatttcaatttcttcttcactcttttcctcaggttcactttcctcttctttttcaagcatttcaccatcattttgctttttttcctcttccaggtccattggtttttccagggctgctttctcttccttttcttcttgctctagtactccttttgtttgtggtatacatatgtcggtttttttatactctgtatctttatgttttttctttacttttcttggccaacaaaatgaagtaattaatgctattggcactcctgctgtcacaagataaatcaaccaaagccatgggtgcccttcagcagctgccattaactgttttaatacaccaggcttattagcatttgctatcattattttccatctccaaccatctgcagcccagtgatctgctacttccttttccgaacagataataaaattatcaaagtagatatcagaggtcatagaccaaagctctaaaccaagagcactgaaagaagtcagaagaaatggatgatcatcttcgaaataatctggattaggaatttttcgaggactccagattccctgatagttaggattatcgaccagtggaggtctccatactcctttgtattttgggttatctatcatgggaggtttccactcaccacacccaatccgacatgctggattaagaatctgaggtgcctcccattctccatccgtgtcttcattccagtcatcaggtttttcagcattaggatcagggataaattttggttcatcatcaagccagccagcaggtttaacaacacttgaatcttctatttgggcaggttcactttcatcccagtcttctggtttgacggcagaaggatcaggaatttttgctctttcatcccattcctcaggttttttatcattgggatcttcaatttctttgggaggtttgataggaggaaccacatcctctaggaggcttcctttgtttacaactgtttgatcaactaacacctcaaatgtgtcatctggattcatcacaagggtataaagatgagtcttcctgtctgtaaagaactttttaaggtctacatctggaggtttggcatgtttctcttcgaaaactccagttttgggatgtttatgtctgaagataaaatgaagtttataatcttctccacatttatctggtccaaacataatgatataggatgttttatcataaaagttttccagaatcaaatcatcagtgtctgctaggagtttaatgtatgcacctccacaatcaataccatcttgaaaatttacttcatattgaactatcaagggtttatcagcaaaaatgaatggttttgctaatacagcagatattgcatgatgctttgctctagattttaataccagtcctctgtcaccaggtacctggttttctttcaactcttcaatttcccatcttccatcgtatattgaaatttcctcatccatgtcatctttctttgcttttgataagacccatccagccaaccttccactatcaaaagtttctgcaaaatatacttctcctataggttgaggtgtcttatatttaatctctgaggaaagttcactttcattaacatcaatttcttctgaattttcttcaaagtcttccgtctcaacatcatcatccataaattctgcattaattgagatgaacagaagacccaaacatagccaaaaggcttggaaatgcatattgattatctctcttgcggcctgttttcggcagtgacagctcagatgtccaagtcgttgccacttggtccccgcgtctcttcagaccagtcccgccggcggccgcgcagcagcgactact

SEQ ID NO: 19128 - RNA, 2109 nt, Homo sapiens
  source 1..2109: mol_type = other RNA
tgggttcctggcatgctgatttttacaatgccaaacatccctctcgggaattaaaaatatttcaatctagtttagtcctttcgtactcttcttttgcgtactgactttatcggcccatctccagatcctgtgctctcatctgcttctttcatctcatcctctgacccagacttatttgattgattactttcttcttgcccttctatgatttcaatttcttcttcactcttttcctcaggttcactttcctcttctttttcaagcatttcaccatcattttgctttttttcctcttccaggtccattggtttttccagggctgctttctcttccttttcttcttgctctagtactccttttgtttgtggtatacatatgtcggtttttttatactctgtatctttatgttttttctttacttttcttggccaacaaaatgaagtaattaatgctattggcactcctgctgtcacaagataaatcaaccaaagccatgggtgcccttcagcagctgccattaactgttttaatacaccaggcttattagcatttgctatcattattttccatctccaaccatctgcagcccagtgatctgctacttccttttccgaacagataataaaattatcaaagtagatatcagaggtcatagaccaaagctctaaaccaagagcactgaaagaagtcagaagaaatggatgatcatcttcgaaataatctggattaggaatttttcgaggactccagattccctgatagttaggattatcgaccagtggaggtctccatactcctttgtattttgggttatctatcatgggaggtttccactcaccacacccaatccgacatgctggattaagaatctgaggtgcctcccattctccatccgtgtcttcattccagtcatcaggtttttcagcattaggatcagggataaattttggttcatcatcaagccagccagcaggtttaacaacacttgaatcttctatttgggcaggttcactttcatcccagtcttctggtttgacggcagaaggatcaggaatttttgctctttcatcccattcctcaggttttttatcattgggatcttcaatttctttgggaggtttgataggaggaaccacatcctctaggaggcttcctttgtttacaactgtttgatcaactaacacctcaaatgtgtcatctggattcatcacaagggtataaagatgagtcttcctgtctgtaaagaactttttaaggtctacatctggaggtttggcatgtttctcttcgaaaactccagttttgggatgtttatgtctgaagataaaatgaagtttataatcttctccacatttatctggtccaaacataatgatataggatgttttatcataaaagttttccagaatcaaatcatcagtgtctgctaggagtttaatgtatgcacctccacaatcaataccatcttgaaaatttacttcatattgaactatcaagggtttatcagcaaaaatgaatggttttgctaatacagcagatattgcatgatgctttgctctagattttaataccagtcctctgtcaccaggtacctggttttctttcaactcttcaatttcccatcttccatcgtatattgaaatttcctcatccatgtcatctttctttgcttttgataagacccatccagccaaccttccactatcaaaagtttctgcaaaatatacttctcctataggttgaggtgtcttatatttaatctctgaggaaagttcactttcattaacatcaatttcttctgaattttcttcaaagtcttccgtctcaacatcatcatccataaattctgcattaattgagatgaacagaagacccaaacatagccaaaaggcttggaaatgcatattgattatcttttctctcccagtcctgagctttggttgccatttgcttttaactcccaagcaaacacctcctctttgttgcttgggcagatgctctcttgcggcctgttttcggcagtgacagctcagatgtccaagtcgttgccacttggtccccgcgtctcttcagaccagtcccgccggcggccgcgcagcagcgactact

SEQ ID NO: 19129 - RNA, 20 nt, Homo sapiens
  source 1..20: mol_type = other RNA
tggtagagctgaggacaaat

SEQ ID NO: 19130 - RNA, 720 nt, Homo sapiens
  source 1..720: mol_type = other RNA
tggtcagaggcagcaggaaatgaatctgtcttctgttcatatctggctgcaaagctcacaaacgctcaagctcaggctgcagcaaggttttgagaagtccagcctcaatcatcttgttttttaatcttcaatcatcttttgagtttccgtcctctacctccagcatcttccagccgcacaccccttctttctagtctccaaacactaagctggcttcccctggagacttcactcttgttccctctgcctggaattctttgaagccagaactttgcaagccccatcctttctcatccttctttattcagctcaagatgtcgccatctcagaaaggcctcccttcaacatccaagcattctctctcccatcaccctgttttttcttcatagctcttcttgcaaagtgcagttatttattacatttttgtttcccctgccaacctgggaactcaatgagggcagcgatcttgtctgacgtggtcgccacggtgttgccagttcctagactaaggcctggcccttggatggcgctcaagaaggagtaagaaattcctttaacttagggaattctggaatcgctttctcccggcagagccgactctaaccaagtgggaaaggcgaggtccgtggctgcctgtggcccaggggtgacggtttggcccaaggccccacctccgccccgcccccggccccgcccctgttcttgtcctcccccacgggt

SEQ ID NO: 19131 - RNA, 903 nt, Homo sapiens
  source 1..903: mol_type = other RNA
tggtcagaggcagcaggaaatgaatctgtcttctgttcatatctggctgcaaagctcacaaacgctcaagctcaggctgcagcaaggttttgagaagtccagcctcaatcatcttgttttttaatcttcaatcatcttttgagtttccgtcctctacctccagctacaggaatgagtccaatgttcagaaaagtgagggtatcagggggcagtagagggggaaggccagcccagagggtaaggacctgagccctggaactgtctgggttaaaatcctggctctgctgctagttgtgtgaggtaggcaagttgctaaaatccccctggatttttagttttctcatcccatcttccagccgcacaccccttctttctagtctccaaacactaagctggcttcccctggagacttcactcttgttccctctgcctggaattctttgaagccagaactttgcaagccccatcctttctcatccttctttattcagctcaagatgtcgccatctcagaaaggcctcccttcaacatccaagcattctctctcccatcaccctgttttttcttcatagctcttcttgcaaagtgcagttatttattacatttttgtttcccctgccaacctgggaactcaatgagggcagcgatcttgtctgacgtggtcgccacggtgttgccagttcctagactaaggcctggcccttggatggcgctcaagaaggagtaagaaattcctttaacttagggaattctggaatcgctttctcccggcagagccgactctaaccaagtgggaaaggcgaggtccgtggctgcctgtggcccaggggtgacggtttggcccaaggccccacctccgccccgcccccggccccgcccctgttcttgtcctcccccacgggt

SEQ ID NO: 19132 - RNA, 169 nt, Homo sapiens
  source 1..169: mol_type = other RNA
tggtctgcaaagagatgactgtttgggggtcagaacggacggagcttggactagcaagccggaatgttccatgaggtcccctcctcgcgttcctcaaacgcgaggtgggggacgaggaagtgcagagccctcccaaaccaccctcctgttctagcacgctcccctcact

SEQ ID NO: 19133 - RNA, 9698 nt, Homo sapiens
  source 1..9698: mol_type = other RNA
tggtctgtctctgccctggcaccccaggaggagggagctctgcacacccatccctgtggctcagacggagcctcctggccactccgtgaccacatccttgcagggtggggccgaagcaatctgaaatgagccacgttgggggtgggtggggagactcagccactgctgtcatgaggcatccgcaaggcatgactttcagcacggcaggagagagcgggagcacattccatctagcctggcttagagacattttgtttgtcctctttttaaaaccgagattaaaatccaacctccatcttcctaggctgtgattttcttttccttccctgaagataaggagttaggaactgttgcttctcaaatgccgcattgctctgggaggccaaaatctacctggaaacatccagctctgttcctttgcacaggtggttctcatgggacagagtccctccgaggcatgggcgctgtcctaagcacagtccagcagcagccaggaggccggcgtagcctcggacaggccgctccgtacagatcaaggtttactaagagtggaggggagacggaaaacatgagcttgaaacagaagtgtcatgatgttgtatcgaaaacccgagagcaacaaacatatctcgaatctgctcatcctcaacctaagacgtctcaacactctccctggcatgtaaagccacatcctcatggctgcagagagcagtcatcagagtgcacagaaagcagcgctggccatggtctccatttatcgcttctcttccaagaaattccagtgctcacatcctggcttcccgcccacttcgccctctccggggccgaggggaaggaggtggcactgtccactgtggtgagtctcatccggggaactgtgggttgcgattctcatgcagaagtggctttgggcagagcatctaggatttttggtttagaatatttccccctccactcagaaaaaggaggagaaaaggaagaaggaataggggagagaggaagggagggagggaaagaagggagggaaggaaggaggaaagagaggaaggaagggagggaaggagggagggagggaggaaagaagagaggaagggaggaaggaaggaaaggaggggtaaaggaaaggaaggaggggaaggaagggaggagagaaaaaaggaaacttgccataccctctaattttggaaagactgaaaaggggttttccagcctatacaaaactctccttggtctcctggggccatactcagcaacgctgacagcacagaatccaggcaatatccacaccctctgcccatggaggtgcacaaaacatctaggtaagcaggggccacactttctgcatgtggccaggagactggctcctgggtggcactggtcagatactgctcagttgtcccctaccctcaggtcactgggggaacggcacctgcccgtttgccgtgcactggggggcactgacagggtggtcttgagtcttgtgtgtgtcacgctgctgctggtgagggggcacttacagggacccggggcacacacgccagtgggcaccagcagtgctcccgttccatccagacccgggacccgggctgaggggtggaccatggcagcccagtcgtctgttgcaaagatgacgtgaggggctggaggcatggccatctctgagctgttaagttttccaaagtagttcatactcttttcatctagctgaaaaatttaaaccaaacaatgacaattttaaataaaaaaaagaaacatttccaaaaaacctgttaaggctaaaagctggcctcggactgggagagggggcagcagcagcgccagtggtggagaagcggtggctgctgcgagcagccagcagaagccaggacagagggaggggacggcctggtgtgcacgaggcgagtcgggagcgtgtgttctcagagctgttttgctttatttgcagacactgttgcttttcatctttcccatgtacaaagctgaacaattaataaaaaggcacctggagacagcaaagacgcattcatttcatgtgacatagtttaaaaaaagataaaaagattttaaaaatactctggttaacaatgcacgcttcctacgtaacaagcaattctggagacgccgtcccgtgtcctcgtgtcccgcggagttgaccgtgtgctgtgttcggggaaggagagggccagcgtggtggcttccagccctaagaggcttccctctccctcgctgtcaggtgagaaggaagggggaaagacaggcagaaaagcctgaggaccgcaccactgcagtgacacagacagtgacggctgagccacaccttagcatccctgcctggccgtcaggaacctgaaagccgactccttgactagacactgccaagtgagaacatttcagaaacagatgaagttgggacaaaacgcactgagcccagggaaaaacgtttgctcttcaaaccccaggagccgccgaggatgtcctgcgttgagaagggtgtgagccgctggttctctggaagaggaggtagaaagagacgggggccggccggggcagctctgagatctcacctgaccctccactccctctccccgcttgacccttcctagttggtcttgaagacggagaaacccagggctggggaggtctgaggtcctcccaggccccggaggtgccaagccattgcaccagtgaaatacaccttctcttaaaaagaaaagaaaaagaaacaaacctgcttcctgcagcgaagttacaaaaagccgtttaaaaaaaccttcctaattgaaatctagtgtccacaagtaggtaaaatcatcacttatcagatttttttctttttaaacaaaaacttcagctcagttattggagttgattgtcttaacaaaaatagactccggaaagttgcctccgttccgccctgagggaggcgcggcgctttgctcacacgaaggaggagaagccggtgagcggagttcgcgcgccggggccagcgggggtgtagacgccgcccgcgctctgcgtggtgatgaccgggtgcagctgcgcgcccgcctcggagcccgccaccgcctcgtacctgtgcggcgcaggtgcgcggccctgggccctgcgcttccatgagttgtagtaggtggggtcgctcatgtagtggttcacgaaggagtgcttgggcagcgcgtcctcgtagtcagagtccgtggcctcagattctgatgcatctgccgacttctccttgaggctcacgctctcggtcagcacggcgccgttgtacttgttgcagatgtcctcgtctgagtagtgcaggccgccggggctaggccggggtggggacctggtcccgttcttcttggagaaggtgctcttgacattgaggtggcggctgctgagctccagggcagcaaatcctccgttgtccagggtcacagactcctccatggtggagatcccctttcctgtgctgcagttcttatacttcttattctgcccgtgcaggacgagggcgaacaccaccagcaggatgacgatcaggctggacagagccatcaccaggaggaaccaccactcctcgtagaatggggcttccacttgagctgacacagccgtggaggggttgctgggctccccgtagcccgcctcattcacagccaccacccggaactcgtaagtcactccttgccggagcttatccaggctgagggtgtaggatgtggcgctccgcgggatgtccttcacaaacatgtcccataagccttcatctgagggccgggcctcgatcacatagcccgtggtaggtgtgtcgccagagtgtccctcagtccactgcagcgtcagttcagaggcggacttggtgaccaggacatctctaggcgagcccggggatccctcggctggcccggctgtgatattggcttggagctcgggcccgtaggtgatggtccgcgcttggacacggaagaaataggtcactcccttggtgaggtcccgcaccttcagccagcgctgccagttccctctcacttccacggtcaccaccttgctcaccccttgtacaggggccaagggctcgtacaccacccgatagccctgcaggatgccgttggccgccgcaggctcgccccaggacacgttgagcgtggtggaggttatttctgagaacgccagaaagctgggggccccaggggcggcctggtgggtgcgcccctgctgggggtcactcttaggtccatctccggcggcgttgaaggctgatatgctgaccaggtacttggtatggctggtcaggttcttcagcctcaccacgggctcggggaggaagaggaccttcattttctccgtttcgttctggctgtctgcctcccagtagtaaatcttgtagccttggatgttcccattctggctctccgggggtggtgggtcccacgtgacctccagctggctggccgtgagtggggtcacctgcacgttctgcggggccatggccggggcagcctcgccgacaaagacctccacgggcgcgctggctgggctctcgccgatgatgttataggcggtcattattacttcatagcgccggtacttctttaaatctgtgagctcagcatgtaaagctatagggtttttgagcgtcttggcctcagtgcctgacccggcttcatactccagctccctgtagtagatcctgtatccctgaagaaggccattcaggctttcgtccctcggaggctgccactgtatcaggacagaggacgtggtgtgtggcgtcgctgagacagatcccgggggctctcctggaacatcctgcagcgtggtcaccgcctctgtctctgaactgaagtcactgtccccaatgtcgttggtggctttcaggcgcagcttgtaggaggtgaagggcctcagtctgtcaacgacgcatgctgtcgcctcatggctgatggacgaggagtaggtctgccactcaccccgaggcagctctcgcacctgcatggtgaagtaccggatgggggaggccccgtcgctgcccgggacccactggagccggaggctgcgtgcggtcacttctgcctggggcaccaggagctctctggggggtgccggccgctctctcttctcggtggtgatgacggtggcctccagtggctccccccagccctgcctcgtcttggcggacagcctgaagatgtatgcggactccggggccaggtcggtggctgtgaactgcctcactgtggcgccgacctccacggtggtgaaggtgtgggggctgctgctggccaggcggtaggcaatctggtaccccaggatgatgccgttgggctcctccggaggttgccacactatccgcacggaggtgagtctcacttcggggaacacgagcctcactggtgggcctggggcatcgtctttggtgcgctccaggatgaggggcgtgctggggaccccgttcccgatgcgggtgaacgccagcacctggagctcgtagagcacgaacttgcgcaggcctgccagcagggccgactgcgtgtggttccctcgcacgatgtggctcctgggctcgggatccaggtctttggcccggaacaggatcttgtagcccagtatgagcccattctggtcctgttccggcacggatgtccatgtcagtaaaatctgggtcgagctgacagcctcggctgacacgttctcaggggcggctgaaggaactgactcccgcgtccggccccgcaccacctcgctccacggcccagccccgacggcgttgaaggcctgcatctgcagctcgtattccatccactcctccagctcctcgatggtgaattctctctccagccggtcactgacgacttgggccactgctgaggactggaggtctgagcgccagtacttaatcctgtagcccacggactcggggttcccgttgtactgagaatccggcaggggcacccagcgaagccgcaggctggtctcactggcagtacggaccgtgacgctggttggagccacgtcgggtggggcctgcagggtctggatgacccgggaagacggactgtaggggctcggcccaacaatgttcacttgcttcattcgaaatctgtagtgagtgtagggtgtgaggtttgggatctccagcatctgggcatcaggctcattctcctcttcatagagggtgacccactcctcctcgtcgccgatagctcccacctgcccctcaacaatccacctggagatggacgttttcccgtcatagcctggccggaactgaagggtggcggagcgagggctgatgttggaaatgaccaggttggatggggcaccaggaaggtctgggggcactccagaagaaatggtggatgaagtcaccaggccagtgcccacggcagtcacagcggccacgtcgatggtgtaggtggtgagagatgagaggccttggatcttgtactcgtgcgtcgtgctgttcagggtgtgcgtgagacgagagtcgttcctgccgtacacttcccaagagatctgatagccagtaatgatgccatttttctccaggggctcctgccagctgaccttgagagatgtgtccaagatctctgtgaaactcagatgtcccacagctcctggtttgtcttcctgagtccagaccagctgaggtgtgctgggaggcccgtccccaggggtggtgaagcacagaacggaagtgaagtaggcggtaaacttcttcaggttcgttatgtgtccatggtggactccgtggaaatctggggcaatagtgaccacagtgacagcctcgggggcatctgccggccatgccagaagcttgtatccctggttgatgccattgataaactgctgaggcggagggttccacaggaactgaatggtggtggagttcacggcttccgtctgcacgttctgcgggggcgcggtgggcactccctgcaaggtgtactcggtcactgccctgctgaagacgcccagaccggccccgttgtacgccgccacctgtatctcatactgtgtccagatgatcaggtctgtcaccaggcagtagttcacctccgggctggtgatgttccgctgctggtactctccgggaaggccagccaggcggtacctgaggatgtatccacgcaacaccccgttgtgctctgtttctgggggtggctgccactggaccataatggactgattagtccgcccactggccactatatttttcgggggagcactgggtggttcttcaggtagcatcaacctgcttgtctcggcgctgtactggcccctgcccacttcattcaccgcgcacacccggaattgataggtacgagccggagtcaggccactcacggtgacgcctgtcatctcagggccaacgtttgacagatgcaccttccatggagagttgttttcagagagctccacgatgtaataaagaataggactgtttccatcaaagggccggacccaagagagcaccacggcgtggctgtgggaagaattagggctgaccaggaggttctgaggtgaatgaggcagttcaatcacttccagccgggccatcctggagtcattccctccttcagaaacaatctcgcagctgtagtcaccgatgtcgcctgaccacgtctggctgatgagaagggacccgtccttctccaccacgatcctagacgtgctcgatggagtcagggccacgttgtccttcttccaaacgtagcggagtgaaacccgggggtcatgtgtggcaccacagtgcagcgtggccgtggtccccttaatcaccacgtggtcctcaggagggtggacgatggacgtccgattccacacagtgagcgtggccgatgcattcagggagccctctgtgttggccgcatagcaggtgtagttgccggcatcctggatgaagacgggcgcgatctgtagaccccccgattcaagaagcatgaacctaggaatccggacagagccactggccagaatgtggttttctcttttccaggtgatggcgggtttgggagccccggacacctcacaccttagaatggctgtcatcccgtcagtaactgtggtgtccactggccgctgggtgaacactggagcgatattggttacatccaggtaggtgtgggtctggatctcccctccttcattgctggcgaagcactggaagattccggagtcctctggacgcagcttctggatgcgcaggcctccgctggcgagcactttgtatcgaggattctggagcctgctgatggagatggcatccttgtaccactggagggtgggaagggggacccccatggcttgacatccgatgtccacagtttcttctacttcagctgaaatccgactctcgggctcagcagtaaaatatggtggctctatgatgaaaagaaaggccgtcgccctggccggttcaaaagcgctccccggcagcgccgcctcgcagacgtatggcccggtgtccgcggacgtcgggttgctgatggtgaggcgtcttccaaagctgtggaggccactggtgattctcactccattcctcttccaggtcacactcaggtcctccacaggcctggcactggctatacattccaaggtggtctcactggatccagccaccacacttctgttgcccgggggaaccacaatggttggggccatggtttcaggtgtgccaacatctcctggtgtatagtgaagcacatgtatcttctgtggatctgatgccctgatgttgtagctctccaggaatatgcactgggcgagaccccggagcatctctgggctgcaaactgaggctcagggttcctttcagtggctggacccagctggtgagcttcttcctgaacctgcaaagcctagaggctttctaagaaggaaagcccactcccccaccacccccggagcctggcaccaaggccctgcagaggctgtcaggagcttccagtacaggcatggatctcacagcttcactcaaacattgtagtcgccagacctcctggctcaggttgttgcagcctccagtcgagaaggcaaaaggggaagctgttaaatttagcaggagccatgcacattttaaaactgttcttaagttacagggagaagtaaattaaattttgtgaaagctttgacttttaataccatcggtagtacattaaaatgttctgaagattatttatgatatatatattttaaaactggtccaactgcaacgatggaaatgcatgaaaagcttcaagcatgaagtacttaaaacactccttgccatatttagaatggggaatctcgggagacattgcttacaaaacttcccatgtctttaggtgactgtattctcgtatcttatacatctctgcagtgcctggccattgggaaaccagcagggacatcacaggcagttcagatgaacttctaattccagtgtaaacctgtaaaatccttaatactggaaaatcagttagacaataaatattccaagtggcaagtgggtggcccaggagccagggtcagataaggtgagggtgggggcaggtgactgggatcacgaaatcaccatcacctggagaaggcagggtaagatgtggagaagagacagatgtgggaccctgggcagatcctgaatgtctgtggagacatctagaatgccatcgtggctgggataatgaactcgaatgccctcactgtttctttatctcttaaccagagctcct

SEQ ID NO: 19134 - RNA, 8559 nt, Homo sapiens
  source 1..8559: mol_type = other RNA
tggtctgtctctgccctggcaccccaggaggagggagctctgcacacccatccctgtggctcagacggagcctcctggccactccgtgaccacatccttgcagggtggggccgaagcaatctgaaatgagccacgttgggggtgggtggggagactcagccactgctgtcatgaggcatccgcaaggcatgactttcagcacggcaggagagagcgggagcacattccatctagcctggcttagagacattttgtttgtcctctttttaaaaccgagattaaaatccaacctccatcttcctaggctgtgattttcttttccttccctgaagataaggagttaggaactgttgcttctcaaatgccgcattgctctgggaggccaaaatctacctggaaacatccagctctgttcctttgcacaggtggttctcatgggacagagtccctccgaggcatgggcgctgtcctaagcacagtccagcagcagccaggaggccggcgtagcctcggacaggccgctccgtacagatcaaggtttactaagagtggaggggagacggaaaacatgagcttgaaacagaagtgtcatgatgttgtatcgaaaacccgagagcaacaaacatatctcgaatctgctcatcctcaacctaagacgtctcaacactctccctggcatgtaaagccacatcctcatggctgcagagagcagtcatcagagtgcacagaaagcagcgctggccatggtctccatttatcgcttctcttccaagaaattccagtgctcacatcctggcttcccgcccacttcgccctctccggggccgaggggaaggaggtggcactgtccactgtggtgagtctcatccggggaactgtgggttgcgattctcatgcagaagtggctttgggcagagcatctaggatttttggtttagaatatttccccctccactcagaaaaaggaggagaaaaggaagaaggaataggggagagaggaagggagggagggaaagaagggagggaaggaaggaggaaagagaggaaggaagggagggaaggagggagggagggaggaaagaagagaggaagggaggaaggaaggaaaggaggggtaaaggaaaggaaggaggggaaggaagggaggagagaaaaaaggaaacttgccataccctctaattttggaaagactgaaaaggggttttccagcctatacaaaactctccttggtctcctggggccatactcagcaacgctgacagcacagaatccaggcaatatccacaccctctgcccatggaggtgcacaaaacatctaggtaagcaggggccacactttctgcatgtggccaggagactggctcctgggtggcactggtcagatactgctcagttgtcccctaccctcaggtcactgggggaacggcacctgcccgtttgccgtgcactggggggcactgacagggtggtcttgagtcttgtgtgtgtcacgctgctgctggtgagggggcacttacagggacccggggcacacacgccagtgggcaccagcagtgctcccgttccatccagacccgggacccgggctgaggggtggaccatggcagcccagtcgtctgttgcaaagatgacgtgaggggctggaggcatggccatctctgagctgttaagttttccaaagtagttcatactcttttcatctagctgaaaaatttaaaccaaacaatgacaattttaaataaaaaaaagaaacatttccaaaaaacctgttaaggctaaaagctggcctcggactgggagagggggcagcagcagcgccagtggtggagaagcggtggctgctgcgagcagccagcagaagccaggacagagggaggggacggcctggtgtgcacgaggcgagtcgggagcgtgtgttctcagagctgttttgctttatttgcagacactgttgcttttcatctttcccatgtacaaagctgaacaattaataaaaaggcacctggagacagcaaagacgcattcatttcatgtgacatagtttaaaaaaagataaaaagattttaaaaatactctggttaacaatgcacgcttcctacgtaacaagcaattctggagacgccgtcccgtgtcctcgtgtcccgcggagttgaccgtgtgctgtgttcggggaaggagagggccagcgtggtggcttccagccctaagaggcttccctctccctcgctgtcaggtgagaaggaagggggaaagacaggcagaaaagcctgaggaccgcaccactgcagtgacacagacagtgacggctgagccacaccttagcatccctgcctggccgtcaggaacctgaaagccgactccttgactagacactgccaagtgagaacatttcagaaacagatgaagttgggacaaaacgcactgagcccagggaaaaacgtttgctcttcaaaccccaggagccgccgaggatgtcctgcgttgagaagggtgtgagccgctggttctctggaagaggaggtagaaagagacgggggccggccggggcagctctgagatctcacctgaccctccactccctctccccgcttgacccttcctagttggtcttgaagacggagaaacccagggctggggaggtctgaggtcctcccaggccccggaggtgccaagccattgcaccagtgaaatacaccttctcttaaaaagaaaagaaaaagaaacaaacctgcttcctgcagcgaagttacaaaaagccgtttaaaaaaaccttcctaattgaaatctagtgtccacaagtaggtaaaatcatcacttatcagatttttttctttttaaacaaaaacttcagctcagttattggagttgattgtcttaacaaaaatagactccggaaagttgcctccgttccgccctgagggaggcgcggcgctttgctcacacgaaggaggagaagccggtgagcggagttcgcgcgccggggccagcgggggtgtagacgccgcccgcgctctgcgtggtgatgaccgggtgcagctgcgcgcccgcctcggagcccgccaccgcctcgtacctgtgcggcgcaggtgcgcggccctgggccctgcgcttccatgagttgtagtaggtggggtcgctcatgtagtggttcacgaaggagtgcttgggcagcgcgtcctcgtagtcagagtccgtggcctcagattctgatgcatctgccgacttctccttgaggctcacgctctcggtcagcacggcgccgttgtacttgttgcagatgtcctcgtctgagtagtgcaggccgccggggctaggccggggtggggacctggtcccgttcttcttggagaaggtgctcttgacattgaggtggcggctgctgagctccagggcagcaaatcctccgttgtccagggtcacagactcctccatggtggagatcccctttcctgtgctgcagttcttatacttcttattctgcccgtgcaggacgagggcgaacaccaccagcaggatgacgatcaggctggacagagccatcaccaggaggaaccaccactcctcgtagaatggggcttccacttgagctgacacagccgtggaggggttgctgggctccccgtagcccgcctcattcacagccaccacccggaactcgtaagtcactccttgccggagcttatccaggctgagggtgtaggatgtggcgctccgcgggatgtccttcacaaacatgtcccataagccttcatctgagggccgggcctcgatcacatagcccgtggtaggtgtgtcgccagagtgtccctcagtccactgcagcgtcagttcagaggcggacttggtgaccaggacatctctaggcgagcccggggatccctcggctggcccggctgtgatattggcttggagctcgggcccgtaggtgatggtccgcgcttggacacggaagaaataggtcactcccttggtgaggtcccgcaccttcagccagcgctgccagttccctctcacttccacggtcaccaccttgctcaccccttgtacaggggccaagggctcgtacaccacccgatagccctgcaggatgccgttggccgccgcaggctcgccccaggacacgttgagcgtggtggaggttatttctgagaacgccagaaagctgggggccccaggggcggcctggtgggtgcgcccctgctgggggtcactcttaggtccatctccggcggcgttgaaggctgatatgctgaccaggtacttggtatggctggtcaggttcttcagcctcaccacgggctcggggaggaagaggaccttcattttctccgtttcgttctggctgtctgcctcccagtagtaaatcttgtagccttggatgttcccattctggctctccgggggtggtgggtcccacgtgacctccagctggctggccgtgagtggggtcacctgcacgttctgcggggccatggccggggcagcctcgccgacaaagacctccacgggcgcgctggctgggctctcgccgatgatgttataggcggtcattattacttcatagcgccggtacttctttaaatgtgttagttcacacatcgtcgatgtggagctgctgttcaccgtcttgaagctgctttgggctactgtgagctcagcatgtaaagctatagggtttttgagcgtcttggcctcagtgcctgacccggcttcatactccagctccctgtagtagatcctgtatccctgaagaaggccattcaggctttcgtccctcggaggctgccactgtatcaggacagaggacgtggtgtgtggcgtcgctgagacagatcccgggggctctcctggaacatcctgcagcgtggtcaccgcctctgtctctgaactgaagtcactgtccccaatgtcgttggtggctttcaggcgcagcttgtaggaggtgaagggcctcagtctgtcaacgacgcatgctgtcgcctcatggctgatggacgaggagtaggtctgccactcaccccgaggcagctctcgcacctgcatggtgaagtaccggatgggggaggccccgtcgctgcccgggacccactggagccggaggctgcgtgcggtcacttctgcctggggcaccaggagctctctggggggtgccggccgctctctcttctcggtggtgatgacggtggcctccagtggctccccccagccctgcctcgtcttggcggacagcctgaagatgtatgcggactccggggccaggtcggtggctgtgaactgcctcactgtggcgccgacctccacggtggtgaaggtgtgggggctgctgctggccaggcggtaggcaatctggtaccccaggatgatgccgttgggctcctccggaggttgccacactatccgcacggaggtgagtctcacttcggggaacacgagcctcactggtgggcctggggcatcgtctttggtgcgctccaggatgaggggcgtgctggggaccccgttcccgatgcgggtgaacgccagcacctggagctcgtagagcacgaacttgcgcaggcctgccagcagggccgactgcgtgtggttccctcgcacgatgtggctcctgggctcgggatccaggtctttggcccggaacaggatcttgtagcccagtatgagcccattctggtcctgttccggcacggatgtccatgtcagtaaaatctgggtcgagctgacagcctcggctgacacgttctcaggggcggctgaaggaactgactcccgcgtccggccccgcaccacctcgctccacggcccagccccgacggcgttgaaggcctgcatctgcagctcgtattccatccactcctccagctcctcgatggtgaattctctctccagccggtcactgacgacttgggccactgctgaggactggaggtctgagcgccagtacttaatcctgtagcccacggactcggggttcccgttgtactgagaatccggcaggggcacccagcgaagccgcaggctggtctcactggcagtacggaccgtgacgctggttggagccacgtcgggtggggcctgcagggtctggatgacccgggaagacggactgtaggggctcggcccaacaatgttcacttgcttcattcgaaatctgtagtgagtgtagggtgtgaggtttgggatctccagcatctgggcatcaggctcattctcctcttcatagagggtgacccactcctcctcgtcgccgatagctcccacctgcccctcaacaatccacctggagatggacgttttcccgtcatagcctggccggaactgaagggtggcggagcgagggctgatgttggaaatgaccaggttggatggggcaccaggaaggtctgggggcactccagaagaaatggtggatgaagtcaccaggccagtgcccacggcagtcacagcggccacgtcgatggtgtaggtggtgagagatgagaggccttggatcttgtactcgtgcgtcgtgctgttcagggtgtgcgtgagacgagagtcgttcctgccgtacacttcccaagagatctgatagccagtaatgatgccatttttctccaggggctcctgccagctgaccttgagagatgtgtccaagatctctgtgaaactcagatgtcccacagctcctggtttgtcttcctgagtccagaccagctgaggtgtgctgggaggcccgtccccaggggtggtgaagcacagaacggaagtgaagtaggcggtaaacttcttcaggttcgttatgtgtccatggtggactccgtggaaatctggggcaatagtgaccacagtgacagcctcgggggcatctgccggccatgccagaagcttgtatccctggttgatgccattgataaactgctgaggcggagggttccacaggaactgaatggtggtggagttcacggcttccgtctgcacgttctgcgggggcgcggtgggcactccctgcaaggtgtactcggtcactgccctgctgaagacgcccagaccggccccgttgtacgccgccacctgtatctcatactgtgtccagatgatcaggtctgtcaccaggcagtagttcacctccgggctggtgatgttccgctgctggtactctccgggaaggccagccaggcggtacctgaggatgtatccacgcaacaccccgttgtgctctgtttctgggggtggctgccactggaccataatggactgattagtccgcccactggccactatatttttcgggggagcactgggtggttcttcaggtagcatcaacctgcttgtctcggcgctgtactggcccctgcccacttcattcaccgcgcacacccggaattgataggtacgagccggagtcaggccactcacggtgacgcctgtcatctcagggccaacgtttgacagatgcaccttccatggagagttgttttcagagagctccacgatgtaataaagaataggactgtttccatcaaagggccggacccaagagagcaccacggcgtggctgtgggaagaattagggctgaccaggaggttctgaggtgaatgaggcagttcaatcacttccagccgggccatcctggagtcattccctccttcagaaacaatctcgcagctgtagtcaccgatgtcgcctgaccacgtctggctgatgagaagggacccgtccttctccaccacgatcctagacgtgctcgatggagtcagggccacgttgtccttcttccaaacgtagcggagtgaaacccgggggtcatgtgtggcaccacagtgcagcgtggccgtggtccccttaatcaccacgtggtcctcaggagggtggacgatggacgtccgattccacacagtgagcgtggccgatgcattcagggagccctctgtgttggccgcatagcaggtgtagttgccggcatcctggatgaagacgggcgcgatctgtagaccccccgattcaagaagcatgaacctaggaatccggacagagccactggccagaatgtggttttctcttttccaggtgatggcgggtttgggagccccggacacctcacaccttagaatggctgtcatcccgtcagtaactgtggtgtccactggccgctgggtgaacactggagcgatattggttacatccaggtaggtgtgggtctggatctcccctccttcattgctggcgaagcactggaagattccggagtcctctggacgcagcttctggatgcgcaggcctccgctggcgagcactttgtatcgaggattctggagcctgctgatggagatggcatccttgtaccactggagggtgggaagggggacccccatggcttgacatccgatgtccacagtttcttctacttcagctgaaatccgactctcgggctcagcagtaaaatatggtggctctatgatgaaaagaaaggccgtcgccctggccggttcaaaagcgctccccggcagcgccgcctcgcagacgtatggcccggtgtccgcggacgtcgggttgctgatggtgaggcgtcttccaaagct

SEQ ID NO: 19135 - RNA, 9758 nt, Homo sapiens
  source 1..9758: mol_type = other RNA
tggtctgtctctgccctggcaccccaggaggagggagctctgcacacccatccctgtggctcagacggagcctcctggccactccgtgaccacatccttgcagggtggggccgaagcaatctgaaatgagccacgttgggggtgggtggggagactcagccactgctgtcatgaggcatccgcaaggcatgactttcagcacggcaggagagagcgggagcacattccatctagcctggcttagagacattttgtttgtcctctttttaaaaccgagattaaaatccaacctccatcttcctaggctgtgattttcttttccttccctgaagataaggagttaggaactgttgcttctcaaatgccgcattgctctgggaggccaaaatctacctggaaacatccagctctgttcctttgcacaggtggttctcatgggacagagtccctccgaggcatgggcgctgtcctaagcacagtccagcagcagccaggaggccggcgtagcctcggacaggccgctccgtacagatcaaggtttactaagagtggaggggagacggaaaacatgagcttgaaacagaagtgtcatgatgttgtatcgaaaacccgagagcaacaaacatatctcgaatctgctcatcctcaacctaagacgtctcaacactctccctggcatgtaaagccacatcctcatggctgcagagagcagtcatcagagtgcacagaaagcagcgctggccatggtctccatttatcgcttctcttccaagaaattccagtgctcacatcctggcttcccgcccacttcgccctctccggggccgaggggaaggaggtggcactgtccactgtggtgagtctcatccggggaactgtgggttgcgattctcatgcagaagtggctttgggcagagcatctaggatttttggtttagaatatttccccctccactcagaaaaaggaggagaaaaggaagaaggaataggggagagaggaagggagggagggaaagaagggagggaaggaaggaggaaagagaggaaggaagggagggaaggagggagggagggaggaaagaagagaggaagggaggaaggaaggaaaggaggggtaaaggaaaggaaggaggggaaggaagggaggagagaaaaaaggaaacttgccataccctctaattttggaaagactgaaaaggggttttccagcctatacaaaactctccttggtctcctggggccatactcagcaacgctgacagcacagaatccaggcaatatccacaccctctgcccatggaggtgcacaaaacatctaggtaagcaggggccacactttctgcatgtggccaggagactggctcctgggtggcactggtcagatactgctcagttgtcccctaccctcaggtcactgggggaacggcacctgcccgtttgccgtgcactggggggcactgacagggtggtcttgagtcttgtgtgtgtcacgctgctgctggtgagggggcacttacagggacccggggcacacacgccagtgggcaccagcagtgctcccgttccatccagacccgggacccgggctgaggggtggaccatggcagcccagtcgtctgttgcaaagatgacgtgaggggctggaggcatggccatctctgagctgttaagttttccaaagtagttcatactcttttcatctagctgaaaaatttaaaccaaacaatgacaattttaaataaaaaaaagaaacatttccaaaaaacctgttaaggctaaaagctggcctcggactgggagagggggcagcagcagcgccagtggtggagaagcggtggctgctgcgagcagccagcagaagccaggacagagggaggggacggcctggtgtgcacgaggcgagtcgggagcgtgtgttctcagagctgttttgctttatttgcagacactgttgcttttcatctttcccatgtacaaagctgaacaattaataaaaaggcacctggagacagcaaagacgcattcatttcatgtgacatagtttaaaaaaagataaaaagattttaaaaatactctggttaacaatgcacgcttcctacgtaacaagcaattctggagacgccgtcccgtgtcctcgtgtcccgcggagttgaccgtgtgctgtgttcggggaaggagagggccagcgtggtggcttccagccctaagaggcttccctctccctcgctgtcaggtgagaaggaagggggaaagacaggcagaaaagcctgaggaccgcaccactgcagtgacacagacagtgacggctgagccacaccttagcatccctgcctggccgtcaggaacctgaaagccgactccttgactagacactgccaagtgagaacatttcagaaacagatgaagttgggacaaaacgcactgagcccagggaaaaacgtttgctcttcaaaccccaggagccgccgaggatgtcctgcgttgagaagggtgtgagccgctggttctctggaagaggaggtagaaagagacgggggccggccggggcagctctgagatctcacctgaccctccactccctctccccgcttgacccttcctagttggtcttgaagacggagaaacccagggctggggaggtctgaggtcctcccaggccccggaggtgccaagccattgcaccagtgaaatacaccttctcttaaaaagaaaagaaaaagaaacaaacctgcttcctgcagcgaagttacaaaaagccgtttaaaaaaaccttcctaattgaaatctagtgtccacaagtaggtaaaatcatcacttatcagatttttttctttttaaacaaaaacttcagctcagttattggagttgattgtcttaacaaaaatagactccggaaagttgcctccgttccgccctgagggaggcgcggcgctttgctcacacgaaggaggagaagccggtgagcggagttcgcgcgccggggccagcgggggtgtagacgccgcccgcgctctgcgtggtgatgaccgggtgcagctgcgcgcccgcctcggagcccgccaccgcctcgtacctgtgcggcgcaggtgcgcggccctgggccctgcgcttccatgagttgtagtaggtggggtcgctcatgtagtggttcacgaaggagtgcttgggcagcgcgtcctcgtagtcagagtccgtggcctcagattctgatgcatctgccgacttctccttgaggctcacgctctcggtcagcacggcgccgttgtacttgttgcagatgtcctcgtctgagtagtgcaggccgccggggctaggccggggtggggacctggtcccgttcttcttggagaaggtgctcttgacattgaggtggcggctgctgagctccagggcagcaaatcctccgttgtccagggtcacagactcctccatggtggagatcccctttcctgtgctgcagttcttatacttcttattctgcccgtgcaggacgagggcgaacaccaccagcaggatgacgatcaggctggacagagccatcaccaggaggaaccaccactcctcgtagaatggggcttccacttgagctgacacagccgtggaggggttgctgggctccccgtagcccgcctcattcacagccaccacccggaactcgtaagtcactccttgccggagcttatccaggctgagggtgtaggatgtggcgctccgcgggatgtccttcacaaacatgtcccataagccttcatctgagggccgggcctcgatcacatagcccgtggtaggtgtgtcgccagagtgtccctcagtccactgcagcgtcagttcagaggcggacttggtgaccaggacatctctaggcgagcccggggatccctcggctggcccggctgtgatattggcttggagctcgggcccgtaggtgatggtccgcgcttggacacggaagaaataggtcactcccttggtgaggtcccgcaccttcagccagcgctgccagttccctctcacttccacggtcaccaccttgctcaccccttgtacaggggccaagggctcgtacaccacccgatagccctgcaggatgccgttggccgccgcaggctcgccccaggacacgttgagcgtggtggaggttatttctgagaacgccagaaagctgggggccccaggggcggcctggtgggtgcgcccctgctgggggtcactcttaggtccatctccggcggcgttgaaggctgatatgctgaccaggtacttggtatggctggtcaggttcttcagcctcaccacgggctcggggaggaagaggaccttcattttctccgtttcgttctggctgtctgcctcccagtagtaaatcttgtagccttggatgttcccattctggctctccgggggtggtgggtcccacgtgacctccagctggctggccgtgagtggggtcacctgcacgttctgcggggccatggccggggcagcctcgccgacaaagacctccacgggcgcgctggctgggctctcgccgatgatgttataggcggtcattattacttcatagcgccggtacttctttaaatgtgttagttcacacatcgtcgatgtggagctgctgttcaccgtcttgaagctgctttgggctgtgagctcagcatgtaaagctatagggtttttgagcgtcttggcctcagtgcctgacccggcttcatactccagctccctgtagtagatcctgtatccctgaagaaggccattcaggctttcgtccctcggaggctgccactgtatcaggacagaggacgtggtgtgtggcgtcgctgagacagatcccgggggctctcctggaacatcctgcagcgtggtcaccgcctctgtctctgaactgaagtcactgtccccaatgtcgttggtggctttcaggcgcagcttgtaggaggtgaagggcctcagtctgtcaacgacgcatgctgtcgcctcatggctgatggacgaggagtaggtctgccactcaccccgaggcagctctcgcacctgcatggtgaagtaccggatgggggaggccccgtcgctgcccgggacccactggagccggaggctgcgtgcggtcacttctgcctggggcaccaggagctctctggggggtgccggccgctctctcttctcggtggtgatgacggtggcctccagtggctccccccagccctgcctcgtcttggcggacagcctgaagatgtatgcggactccggggccaggtcggtggctgtgaactgcctcactgtggcgccgacctccacggtggtgaaggtgtgggggctgctgctggccaggcggtaggcaatctggtaccccaggatgatgccgttgggctcctccggaggttgccacactatccgcacggaggtgagtctcacttcggggaacacgagcctcactggtgggcctggggcatcgtctttggtgcgctccaggatgaggggcgtgctggggaccccgttcccgatgcgggtgaacgccagcacctggagctcgtagagcacgaacttgcgcaggcctgccagcagggccgactgcgtgtggttccctcgcacgatgtggctcctgggctcgggatccaggtctttggcccggaacaggatcttgtagcccagtatgagcccattctggtcctgttccggcacggatgtccatgtcagtaaaatctgggtcgagctgacagcctcggctgacacgttctcaggggcggctgaaggaactgactcccgcgtccggccccgcaccacctcgctccacggcccagccccgacggcgttgaaggcctgcatctgcagctcgtattccatccactcctccagctcctcgatggtgaattctctctccagccggtcactgacgacttgggccactgctgaggactggaggtctgagcgccagtacttaatcctgtagcccacggactcggggttcccgttgtactgagaatccggcaggggcacccagcgaagccgcaggctggtctcactggcagtacggaccgtgacgctggttggagccacgtcgggtggggcctgcagggtctggatgacccgggaagacggactgtaggggctcggcccaacaatgttcacttgcttcattcgaaatctgtagtgagtgtagggtgtgaggtttgggatctccagcatctgggcatcaggctcattctcctcttcatagagggtgacccactcctcctcgtcgccgatagctcccacctgcccctcaacaatccacctggagatggacgttttcccgtcatagcctggccggaactgaagggtggcggagcgagggctgatgttggaaatgaccaggttggatggggcaccaggaaggtctgggggcactccagaagaaatggtggatgaagtcaccaggccagtgcccacggcagtcacagcggccacgtcgatggtgtaggtggtgagagatgagaggccttggatcttgtactcgtgcgtcgtgctgttcagggtgtgcgtgagacgagagtcgttcctgccgtacacttcccaagagatctgatagccagtaatgatgccatttttctccaggggctcctgccagctgaccttgagagatgtgtccaagatctctgtgaaactcagatgtcccacagctcctggtttgtcttcctgagtccagaccagctgaggtgtgctgggaggcccgtccccaggggtggtgaagcacagaacggaagtgaagtaggcggtaaacttcttcaggttcgttatgtgtccatggtggactccgtggaaatctggggcaatagtgaccacagtgacagcctcgggggcatctgccggccatgccagaagcttgtatccctggttgatgccattgataaactgctgaggcggagggttccacaggaactgaatggtggtggagttcacggcttccgtctgcacgttctgcgggggcgcggtgggcactccctgcaaggtgtactcggtcactgccctgctgaagacgcccagaccggccccgttgtacgccgccacctgtatctcatactgtgtccagatgatcaggtctgtcaccaggcagtagttcacctccgggctggtgatgttccgctgctggtactctccgggaaggccagccaggcggtacctgaggatgtatccacgcaacaccccgttgtgctctgtttctgggggtggctgccactggaccataatggactgattagtccgcccactggccactatatttttcgggggagcactgggtggttcttcaggtagcatcaacctgcttgtctcggcgctgtactggcccctgcccacttcattcaccgcgcacacccggaattgataggtacgagccggagtcaggccactcacggtgacgcctgtcatctcagggccaacgtttgacagatgcaccttccatggagagttgttttcagagagctccacgatgtaataaagaataggactgtttccatcaaagggccggacccaagagagcaccacggcgtggctgtgggaagaattagggctgaccaggaggttctgaggtgaatgaggcagttcaatcacttccagccgggccatcctggagtcattccctccttcagaaacaatctcgcagctgtagtcaccgatgtcgcctgaccacgtctggctgatgagaagggacccgtccttctccaccacgatcctagacgtgctcgatggagtcagggccacgttgtccttcttccaaacgtagcggagtgaaacccgggggtcatgtgtggcaccacagtgcagcgtggccgtggtccccttaatcaccacgtggtcctcaggagggtggacgatggacgtccgattccacacagtgagcgtggccgatgcattcagggagccctctgtgttggccgcatagcaggtgtagttgccggcatcctggatgaagacgggcgcgatctgtagaccccccgattcaagaagcatgaacctaggaatccggacagagccactggccagaatgtggttttctcttttccaggtgatggcgggtttgggagccccggacacctcacaccttagaatggctgtcatcccgtcagtaactgtggtgtccactggccgctgggtgaacactggagcgatattggttacatccaggtaggtgtgggtctggatctcccctccttcattgctggcgaagcactggaagattccggagtcctctggacgcagcttctggatgcgcaggcctccgctggcgagcactttgtatcgaggattctggagcctgctgatggagatggcatccttgtaccactggagggtgggaagggggacccccatggcttgacatccgatgtccacagtttcttctacttcagctgaaatccgactctcgggctcagcagtaaaatatggtggctctatgatgaaaagaaaggccgtcgccctggccggttcaaaagcgctccccggcagcgccgcctcgcagacgtatggcccggtgtccgcggacgtcgggttgctgatggtgaggcgtcttccaaagctgtggaggccactggtgattctcactccattcctcttccaggtcacactcaggtcctccacaggcctggcactggctatacattccaaggtggtctcactggatccagccaccacacttctgttgcccgggggaaccacaatggttggggccatggtttcaggtgtgccaacatctcctggtgtatagtgaagcacatgtatcttctgtggatctgatgccctgatgttgtagctctccaggaatatgcactgggcgagaccccggagcatctctgggctgcaaactgaggctcagggttcctttcagtggctggacccagctggtgagcttcttcctgaacctgcaaagcctagaggctttctaagaaggaaagcccactcccccaccacccccggagcctggcaccaaggccctgcagaggctgtcaggagcttccagtacaggcatggatctcacagcttcactcaaacattgtagtcgccagacctcctggctcaggttgttgcagcctccagtcgagaaggcaaaaggggaagctgttaaatttagcaggagccatgcacattttaaaactgttcttaagttacagggagaagtaaattaaattttgtgaaagctttgacttttaataccatcggtagtacattaaaatgttctgaagattatttatgatatatatattttaaaactggtccaactgcaacgatggaaatgcatgaaaagcttcaagcatgaagtacttaaaacactccttgccatatttagaatggggaatctcgggagacattgcttacaaaacttcccatgtctttaggtgactgtattctcgtatcttatacatctctgcagtgcctggccattgggaaaccagcagggacatcacaggcagttcagatgaacttctaattccagtgtaaacctgtaaaatccttaatactggaaaatcagttagacaataaatattccaagtggcaagtgggtggcccaggagccagggtcagataaggtgagggtgggggcaggtgactgggatcacgaaatcaccatcacctggagaaggcagggtaagatgtggagaagagacagatgtgggaccctgggcagatcctgaatgtctgtggagacatctagaatgccatcgtggctgggataatgaactcgaatgccctcactgtttctttatctcttaaccagagctcct

SEQ ID NO: 19136 - RNA, 9914 nt, Homo sapiens
  source 1..9914: mol_type = other RNA
tggtctgtctctgccctggcaccccaggaggagggagctctgcacacccatccctgtggctcagacggagcctcctggccactccgtgaccacatccttgcagggtggggccgaagcaatctgaaatgagccacgttgggggtgggtggggagactcagccactgctgtcatgaggcatccgcaaggcatgactttcagcacggcaggagagagcgggagcacattccatctagcctggcttagagacattttgtttgtcctctttttaaaaccgagattaaaatccaacctccatcttcctaggctgtgattttcttttccttccctgaagataaggagttaggaactgttgcttctcaaatgccgcattgctctgggaggccaaaatctacctggaaacatccagctctgttcctttgcacaggtggttctcatgggacagagtccctccgaggcatgggcgctgtcctaagcacagtccagcagcagccaggaggccggcgtagcctcggacaggccgctccgtacagatcaaggtttactaagagtggaggggagacggaaaacatgagcttgaaacagaagtgtcatgatgttgtatcgaaaacccgagagcaacaaacatatctcgaatctgctcatcctcaacctaagacgtctcaacactctccctggcatgtaaagccacatcctcatggctgcagagagcagtcatcagagtgcacagaaagcagcgctggccatggtctccatttatcgcttctcttccaagaaattccagtgctcacatcctggcttcccgcccacttcgccctctccggggccgaggggaaggaggtggcactgtccactgtggtgagtctcatccggggaactgtgggttgcgattctcatgcagaagtggctttgggcagagcatctaggatttttggtttagaatatttccccctccactcagaaaaaggaggagaaaaggaagaaggaataggggagagaggaagggagggagggaaagaagggagggaaggaaggaggaaagagaggaaggaagggagggaaggagggagggagggaggaaagaagagaggaagggaggaaggaaggaaaggaggggtaaaggaaaggaaggaggggaaggaagggaggagagaaaaaaggaaacttgccataccctctaattttggaaagactgaaaaggggttttccagcctatacaaaactctccttggtctcctggggccatactcagcaacgctgacagcacagaatccaggcaatatccacaccctctgcccatggaggtgcacaaaacatctaggtaagcaggggccacactttctgcatgtggccaggagactggctcctgggtggcactggtcagatactgctcagttgtcccctaccctcaggtcactgggggaacggcacctgcccgtttgccgtgcactggggggcactgacagggtggtcttgagtcttgtgtgtgtcacgctgctgctggtgagggggcacttacagggacccggggcacacacgccagtgggcaccagcagtgctcccgttccatccagacccgggacccgggctgaggggtggaccatggcagcccagtcgtctgttgcaaagatgacgtgaggggctggaggcatggccatctctgagctgttaagttttccaaagtagttcatactcttttcatctagctgaaaaatttaaaccaaacaatgacaattttaaataaaaaaaagaaacatttccaaaaaacctgttaaggctaaaagctggcctcggactgggagagggggcagcagcagcgccagtggtggagaagcggtggctgctgcgagcagccagcagaagccaggacagagggaggggacggcctggtgtgcacgaggcgagtcgggagcgtgtgttctcagagctgttttgctttatttgcagacactgttgcttttcatctttcccatgtacaaagctgaacaattaataaaaaggcacctggagacagcaaagacgcattcatttcatgtgacatagtttaaaaaaagataaaaagattttaaaaatactctggttaacaatgcacgcttcctacgtaacaagcaattctggagacgccgtcccgtgtcctcgtgtcccgcggagttgaccgtgtgctgtgttcggggaaggagagggccagcgtggtggcttccagccctaagaggcttccctctccctcgctgtcaggtgagaaggaagggggaaagacaggcagaaaagcctgaggaccgcaccactgcagtgacacagacagtgacggctgagccacaccttagcatccctgcctggccgtcaggaacctgaaagccgactccttgactagacactgccaagtgagaacatttcagaaacagatgaagttgggacaaaacgcactgagcccagggaaaaacgtttgctcttcaaaccccaggagccgccgaggatgtcctgcgttgagaagggtgtgagccgctggttctctggaagaggaggtagaaagagacgggggccggccggggcagctctgagatctcacctgaccctccactccctctccccgcttgacccttcctagttggtcttgaagacggagaaacccagggctggggaggtctgaggtcctcccaggccccggaggtgccaagccattgcaccagtgaaatacaccttctcttaaaaagaaaagaaaaagaaacaaacctgcttcctgcagcgaagttacaaaaagccgtttaaaaaaaccttcctaattgaaatctagtgtccacaagtaggtaaaatcatcacttatcagatttttttctttttaaacaaaaacttcagctcagttattggagttgattgtcttaacaaaaatagactccggaaagttgcctccgttccgccctgagggaggcgcggcgctttgctcacacgaaggaggagaagccggtgagcggagttcgcgcgccggggccagcgggggtgtagacgccgcccgcgctctgcgtggtgatgaccgggtgcagctgcgcgcccgcctcggagcccgccaccgcctcgtacctgtgcggcgcaggtgcgcggccctgggccctgcgcttccatgagttgtagtaggtggggtcgctcatgtagtggttcacgaaggagtgcttgggcagcgcgtcctcgtagtcagagtccgtggcctcagattctgatgcatctgccgacttctccttgaggctcacgctctcggtcagcacggcgccgttgtacttgttgcagatgtcctcgtctgagtagtgcaggccgccggggctaggccggggtggggacctggtcccgttcttcttggagaaggtgctcttgacattgaggtggcggctgctgagctccagggcagcaaatcctccgttgtccagggtcacagactcctccatggtggagatcccctttcctgtgctgcagttcttatacttcttattctgcccgtgcaggacgagggcgaacaccaccagcaggatgacgatcaggctggacagagccatcaccaggaggaaccaccactcctcgtagaatggggcttccacttgagctgacacagccgtggaggggttgctgggctccccgtagcccgcctcattcacagccaccacccggaactcgtaagtcactccttgccggagcttatccaggctgagggtgtaggatgtggcgctccgcgggatgtccttcacaaacatgtcccataagccttcatctgagggccgggcctcgatcacatagcccgtggtaggtgtgtcgccagagtgtccctcagtccactgcagcgtcagttcagaggcggacttggtgaccaggacatctctaggcgagcccggggatccctcggctggcccggctgtgatattggcttggagctcgggcccgtaggtgatggtccgcgcttggacacggaagaaataggtcactcccttggtgaggtcccgcaccttcagccagcgctgccagttccctctcacttccacggtcaccaccttgctcaccccttgtacaggggccaagggctcgtacaccacccgatagccctgcaggatgccgttggccgccgcaggctcgccccaggacacgttgagcgtggtggaggttatttctgagaacgccagaaagctgggggccccaggggcggcctggtgggtgcgcccctgctgggggtcactcttaggtccatctccggcggcgttgaaggctgatatgctgaccaggtacttggtatggctggtcaggttcttcagcctcaccacgggctcggggaggaagaggaccttcattttctccgtttcgttctggctgtctgcctcccagtagtaaatcttgtagccttggatgttcccattctggctctccgggggtggtgggtcccacgtgacctccagctggctggccgtgagtggggtcacctgcacgttctgcggggccatggccggggcagcctcgccgacaaagacctccacgggcgcgctggctgggctctcgccgatgatgttataggcggtcattattacttcatagcgccggtacttctttaaatgtgttagttcacacatcgtcgatgtggagctgctgttcaccgtcttgaagctgctttgggctgtgagctcagcatgtaaagctatagggtttttgagcgtcttggcctcagtgcctgacccggcttcatactccagctccctgtagtagatcctgtatccctgaagaaggccattcaggctttcgtccctcggaggctgccactgtatcaggacagaggacgtggtgtgtggcgtcgctgagacagatcccgggggctctcctggaacatcctgcagcgtggtcaccgcctctgtctctgaactgaagtcactgtccccaatgtcgttggtggctttcaggcgcagcttgtaggaggtgaagggcctcagtctgtcaacgacgcatgctgtcgcctcatggctgatggacgaggagtaggtctgccactcaccccgaggcagctctcgcacctgcatggtgaagtaccggatgggggaggccccgtcgctgcccgggacccactggagccggaggctgcgtgcggtcacttctgcctggggcaccaggagctctctggggggtgccggccgctctctcttctcggtggtgatgacggtggcctccagtggctccccccagccctgcctcgtcttggcggacagcctgaagatgtatgcggactccggggccaggtcggtggctgtgaactgcctcactgtggcgccgacctccacggtggtgaaggtgtgggggctgctgctggccaggcggtaggcaatctggtaccccaggatgatgccgttgggctcctccggaggttgccacactatccgcacggaggtgagtctcacttcggggaacacgagcctcactggtgggcctggggcatcgtctttggtgcgctccaggatgaggggcgtgctggggaccccgttcccgatgcgggtgaacgccagcacctggagctcgtagagcacgaacttgcgcaggcctgccagcagggccgactgcgtgtggttccctcgcacgatgtggctcctgggctcgggatccaggtctttggcccggaacaggatcttgtagcccagtatgagcccattctggtcctgttccggcacggatgtccatgtcagtaaaatctgggtcgagctgacagcctcggctgacacgttctcaggggcggctgaaggaactgactcccgcgtccggccccgcaccacctcgctccacggcccagccccgacggcgttgaaggcctgcatctgcagctcgtattccatccactcctccagctcctcgatggtgaattctctctccagccggtcactgacgacttgggccactgctgaggactggaggtctgagcgccagtacttaatcctgtagcccacggactcggggttcccgttgtactgagaatccggcaggggcacccagcgaagccgcaggctggtctcactggcagtacggaccgtgacgctggttggagccacgtcgggtggggcctgcagggtctggatgacccgggaagacggactgtaggggctcggcccaacaatgttcacttgcttcattcgaaatctgtagtgagtgtagggtgtgaggtttgggatctccagcatctgggcatcaggctcattctcctcttcatagagggtgacccactcctcctcgtcgccgatagctcccacctgcccctcaacaatccacctggagatggacgttttcccgtcatagcctggccggaactgaagggtggcggagcgagggctgatgttggaaatgaccaggttggatggggcaccaggaaggtctgggggcactccagaagaaatggtggatgaagtcaccaggccagtgcccacggcagtcacagcggccacgtcgatggtgtaggtggtgagagatgagaggccttggatcttgtactcgtgcgtcgtgctgttcagggtgtgcgtgagacgagagtcgttcctgccgtacacttcccaagagatctgatagccagtaatgatgccatttttctccaggggctcctgccagctgaccttgagagatgtgtccaagatctctgtgaaactcagatgtcccacagctcctggtttgtcttcctgagtccagaccagctgaggtgtgctgggaggcccgtccccaggggtggtgaagcacagaacggaagtgaagtaggcggtaaacttcttcaggttcgttatgtgtccatggtggactccgtggaaatctggggcaatagtgaccacagtgacagcctcgggggcatctgccggccatgccagaagcttgtatccctggttgatgccattgataaactgctgaggcggagggttccacaggaactgaatggtggtggagttcacggcttccgtctgcacgttctgcgggggcgcggtgggcactccctgcaaggtgtactcggtcactgccctgctgaagacgcccagaccggccccgttgtacgccgccacctgtatctcatactgtgtccagatgatcaggtctgtcaccaggcagtagttcacctccgggctggtgatgttccgctgctggtactctccgggaaggccagccaggcggtacctgaggatgtatccacgcaacaccccgttgtgctctgtttctgggggtggctgccactggaccataatggactgattagtccgcccactggccactatatttttcgggggagcactgggtggttcttcaggtagcatcaacctgcttgtctcggcgctgtactggcccctgcccacttcattcaccgcgcacacccggaattgataggtacgagccggagtcaggccactcacggtgacgcctgtcatctcagggccaacgtttgacagatgcaccttccatggagagttgttttcagagagctccacgatgtaataaagaataggactgtttccatcaaagggccggacccaagagagcaccacggcgtggctgtgggaagaattagggctgaccaggaggttctgaggtgaatgaggcagttcaatcacttccagccgggccatcctggagtcattccctccttcagaaacaatctcgcagctgtagtcaccgatgtcgcctgaccacgtctggctgatgagaagggacccgtccttctccaccacgatcctagacgtgctcgatggagtcagggccacgttgtccttcttccaaacgtagcggagtgaaacccgggggtcatgtgtggcaccacagtgcagcgtggccgtggtccccttaatcaccacgtggtcctcaggagggtggacgatggacgtccgattccacacagtgagcgtggccgatgcattcagggagccctctgtgttggccgcatagcaggtgtagttgccggcatcctggatgaagacgggcgcgatctgtagaccccccgattcaagaagcatgaacctaggaatccggacagagccactggccagaatgtggttttctcttttccaggtgatggcgggtttgggagccccggacacctcacaccttagaatggctgtcatcccgtcagtaactgtggtgtccactggccgctgggtgaacactggagcgatattggttacatccaggtaggtgtgggtctggatctcccctccttcattgctggcgaagcactggaagattccggagtcctctggacgcagcttctggatgcgcaggcctccgctggcgagcactttgtatcgaggattctggagcctgctgatggagatggcatccttgtaccactggagggtgggaagggggacccccatggcttgacatccgatgtccacagtttcttctacttcagctgaaatccgactctcgggctcagcagtaaaatatggtggctctatgatgaaaagaaaggccgtcgccctggccggttcaaaagcgctccccggcagcgccgcctcgcagacgtatggcccggtgtccgcggacgtcgggttgctgatggtgaggcgtcttccaaagctgtggaggccactggtgattctcactccattcctcttccaggtcacactcaggtcctccacaggcctggcactggctatacattccaaggtggtctcactggatccagccaccacacttctgttgcccgggggaaccacaatggttggggccatggtttcaggtgtgccaacatctcttgctatgctcaaatgaatgaatgggcttgtcttgttttctccatttttctcattcacggcctgcacgtagtatgccccggcatcactggttgtggtggcgaggatcaccagctgattctccaatgtgatggctattctgttgcttggaataatcttgtgcccttctctaaaccaagtcacttgaggtctggggtagctggtgatgggcagcaggtttagaatcgctgcacgtccttgagaaactgttttcctctggtccgtatccatgaaacttcccatatatgcgacttgaacttctgattttctttgcaggagtgctcccattctgtttcgcaccacgcagcggtaaaacccagcatcgagcttctgcaaagatggaataatgtacttatattcgctgctgtaggtggtgagctcactgtcatcgcgcatccacttgaactccaaaggccagctcccttcggcaaggcaggtgagaacaaggcggttcccttccaggtggatctgtggtaggcctggctccgttttaaaatatggagcaacatcatcttgcgccagcgcccggagcaagtgcagctgcagcgccagcagcgcccaccagccgcggcggcccggccccaactttgccgcccgccgcccgccgcaccgccccgcgcccgccgtgtccccgccggaggtctcgggcgccgcccggggtcgcgagggctccgggccggggcgcggcgccagcgaggggcgggcgcggccgggcggggatccccgcggccgcccggggcccgcgcgctcagggggctccgcgccgccgccgccgccaccggccgccgagggccgggcgccccgggccatgccgagcagccgccaccccgagcgccgcgccggacggacgggcgggcaggacaggcgggacggctccgagcgggcgcggccactccgcgggaggcgcggcgccccccggcccgaggtgagcggccgcccagcgctgaggggcggcgtcctgggtccccgcgtgaggggcgcggcgcgggccggggacgagccgggcgagaagaagttgtcaacgggggaaattcgcgtccggcgctcacgcagtcccgagcccgccgcgctagctccgaggggtccgccgggcgcggaggagccgccgccgccgccgcccccgcccggcgctgagaagaaagtgc

SEQ ID NO: 19137 - RNA, 267 nt, Homo sapiens
  source 1..267: mol_type = other RNA
tggtctgtctctgccctggcactcaattttttcttctagtcttaactcctcctccttccctctcaaaatgtattctgcacagaaagccactcctattcctcacctccaagccaaattatacagtcctctccaggaacactgacatactcagaaacctcccctaatccatctcaccttaggctgctctttccccacctctggctcctgtcacactatataaaatctttttttttttttttgagacagccttgctgtcacccaggctgg

SEQ ID NO: 19138 - RNA, 451 nt, Homo sapiens
  source 1..451: mol_type = other RNA
tggtctgttcattctctctttttggccacctcactgcaaagttgagttcactgatattgcagacagagggggaataaagagggggaagtagtgaaagaaaagagagggaaattaaatctgttttagctttaccaagggaaaattttcacattataaaaccgtccgttcacatccctgcgccgctcactgactgcccatctggtactacgcgacacaaaataatgatgcagccagaaacgatgtcctgggtcgtttcattttccagccatatgcctccaagctttcgggatatcctgggttgtcagaaataatctctggtcagtgaaagaggagttcggtcgtgtgcatggacccataaaaaagagctagttagcttagcaggagtttaacggcttccttgatgcagcaaaaatgtccttcttcccatttaggctgtttgatccaagtcatt

SEQ ID NO: 19139 - RNA, 477 nt, Homo sapiens
  source 1..477: mol_type = other RNA
tggtctgttcattctctctttttggccacctcactgcaaagttgagttcactgatattgcagacagagggggaataaagagggggaagtagtgaaagaaaagagagggaaattaaatctgttttagctttaccaagggaaaattttcacattataaaaccgtccgttcacatccctgcgccgctcactgactgcccatctggtactacgcgacacaaaataatgatgcagccagaaacgatgtcctgggtcgtttcattttccagccatatgcctccaagctttcgggatatcctgggttgtcagaaataatctctggtcagtgaaagaggagttcggtcgtgtgcatggacccataaaaaagagctagttagcttagcaggagtttaacggcttccttgatgcagcaaaaatgtccttcttcccatttaggctgtttgatccaagtcattgtgttcctctgagcctcggaaacttt

SEQ ID NO: 19140 - RNA, 694 nt, Homo sapiens
  source 1..694: mol_type = other RNA
tggtctgttcattctctctttttggccagtcagaagaatgatatctcatttgaattatccaaggagagagaggatggaggacgcgtttcctcaatcatgaatcacactgactccacagccacgtgggcactccagcccaagtctcacacaccaacacaggtgcgaggagcgctggtgccagtcatccagcgcctgggggccagagcggctccgaggatcctcttcagcacctggctagggaagtggaggcagcagctgcagccgccccctgccacttccccagagccgccccctactcgctgagttccagaatgggggcaccggcttgggggccacgagcacggtccccgagcgcgcggccaaccggtgggtgggcaggttcgcgcccagcagagacgaccctcgaggtggcaaagttgggtgtccaagccagctccgcggggcagtcctgggtgggagaagggagcgtcccgggatgagcgacactggccgggccgcccctgcacggggaaggtggagggccggggctgcagcgggccaagggccgcggctggcctgaggctgcgaagcccacccgcggcgggaaagcagcgctcgggagcgggctcagggagagcagccgccaccggcgccgccttcccggcaagtagatcggcgcggggcgagcgggcgcggagagcgcggggcggagagc

SEQ ID NO: 19141 - RNA, 839 nt, Homo sapiens
  source 1..839: mol_type = other RNA
tggtctgttcattctctctttttggccagtcagaagaatgatatctcatttgaattatccaccgccatgcagcagagaaggagaatcacataattttaaaattcaggctgagggccactgtggacgcagaaggctgacttccgaccacctgcttccccactagacttgttccaaatggctttcttgagaggtgattcacaagtgcaaggagagagaggatggaggacgcgtttcctcaatcatgaatcacactgactccacagccacgtgggcactccagcccaagtctcacacaccaacacaggtgcgaggagcgctggtgccagtcatccagcgcctgggggccagagcggctccgaggatcctcttcagcacctggctagggaagtggaggcagcagctgcagccgccccctgccacttccccagagccgccccctactcgctgagttccagaatgggggcaccggcttgggggccacgagcacggtccccgagcgcgcggccaaccggtgggtgggcaggttcgcgcccagcagagacgaccctcgaggtggcaaagttgggtgtccaagccagctccgcggggcagtcctgggtgggagaagggagcgtcccgggatgagcgacactggccgggccgcccctgcacggggaaggtggagggccggggctgcagcgggccaagggccgcggctggcctgaggctgcgaagcccacccgcggcgggaaagcagcgctcgggagcgggctcagggagagcagccgccaccggcgccgccttcccggcaagtagatcggcgcggggcgagcgggcgcggagagcgcggggcggagagc

SEQ ID NO: 19142 - RNA, 1317 nt, Homo sapiens
  source 1..1317: mol_type = other RNA
tggtgggtggggaggagaagtgcagatctttctacaaagtctatctgaatctctgatgacagaaaggaacattgaaatttgaaaaatactctaaaattggagttgccttcattattttctagtcagtaaatatttaagttgccttgatatttaaattaatagttttttttaagtatgaaatttagacaatttactcataggagaaatgggccaaaaatgtacaagaatgttggggtctttcaaaatgcaagagttgaagaataaaattgtggtacaaggaggagagtagtgaaatgaaatgatccgagaatgggaggaggagggactgggaaaagggagcggggaccctcctggcacaggcagcatgctaccctgtagctgctcatccatcaccaaagcccctgcctgttcatggtaatctggcaagcaatgaaatacctccctgcttcccacgtctccctctaccatgtctcaatatgtcttgaagtccaccattagcacctctatcctttaagtctcagctgactcctccatcaaataggtggcatttatgttgggattttaggactgcaaatgtgtctagttttgcagttctggaactttctagaatcacacattaggtgggctagataagtagtttctctagttttgtgctcttgcaactttttatgtaattgcattgattattccttgattacttcttaggagaatccagacagagcccaggtaagcaactaaaatacctatgccctttgtccttctgagatgcagtaggaaaccacctgtcagggtaattcccacatttcatgttactgggctgctcccctggacatgaggggggatggttctaggcccaggtgcccagcaagccttgtgctcctttctatcatggcttttctctcccagagctggtcaactccagggcttaaagcaagtaagccaatgtcagcacagagaagatgtgcagtgaagtgctgcccacgtgacggccagggccaaagctcaggccttctgccgtgtaatctcgggcaagttccctaaactcaagttatttgaacaggaatgcaaatggggtgagaataagggtctggagacaagggtccccgggttcataccctggctccatcacttgccagaaccatatgcatgaggcttaacttccagtctgtccttttctttgtctgtaaaatggaacttataatagcatccacatcttagggctgctttgagttaatctgataagttaatgcatgtaaaatgcttacaaattgccttgttcatagtacttaataaatatttgacattttaggccgggca

SEQ ID NO: 19143 - RNA, 2338 nt, Homo sapiens
  source 1..2338: mol_type = other RNA
tgtaggcatgaggcagggcccaggactcttaatcatctacaagctcaacaggtgactctattgtgcacctgggtttaagaactacaaatctagaaaacatactttaaacccactagagtaagtcctagctcttcactttaatatacatatactaacatggacatctccagtgaaaaacactaggggataaatatctcatttatgtaaataattgttcttaggctctgtctgggcttgggttctcaattaatctactgttccttcctacatcataaataatccgttatgcttaagttacctactgcataatgactcctctgtgtttctcagggtgatcacttgaataatctgctggaaccttaacctctaattccagacattaacaaattaaggcagttaacgttataaataaacctcatagcaccttattaagctgccggtgaaagagcatgagtagatattgaaggtgacttgcaaatcttaaatgttcacacaaatgggtatagtgtttgttcaggatgatggaaaagctgtagaaatggaaagtggtgatggttgcctaacactgaatgtacctaataccaccaaactgtacacctaaaaacggttaaatggaaaattttatgttatgtatgttttatcacaataaaagaaagtccacccagacaattcttaataaatatataatgtgctgcttagcttattctcgaaaataacctctaactaactctgggaatactggacctcaagctatatataccttctaatattactgcatttaaatattttgcattaaatcattctttaaatgtaattatggttacagtgaatgagtatcactatagtaaacaagttactaccttcacctaatcctcataaaaaccccaagagacagaaattattactctcattgcacatacaaaaaaaatctgaaagcttaatttgtcaaaggctatattgctagcatgtggtaaggctgaagttcactcatgggtctgtgcacatcgttataatatgaactaactggggcctgaaaatatttttgtagtgaagaaatctcttagctgttacactttttgtgacaacaagaatgaaccagtaaatagttttatttcctctagattgtaaactacaagagaggaatagccacagctaaatggaactgtaaattttacagattacaatggggattaggaagggaaggaggaggcagcaccaatgattaccagatccacaactttagctcttatctctcgcttgagattcagatctatattttcaacattttgagctctgtacagtaaaaaagaggagcaaaccaaggtcagatactagagggcaaagcaggggcaagatgcccaaacttgggctatgggacaaaagtggacataaatttaggccaccttagtggcagtctgctcgttcatgcagcctgtgtccaaatctccactctgtcagcctgcattgaacccacacatgtatatatacatatatgaaatagatgcgtgaatcttattggttctgtccctcaggagaaccctaatgcaagttacatgaaaaaatgctcaaactagtaataagggaaattcaaattaaaactttggcaaaatgccatttcacacctatctgattgacattaaatattgatgaggattagtaagcttatggagcaataaaaatttatgaattgctaaaggtcattgaaattggtacaagcattttagaaaaacaattttatattactcaatacagttgaaaataacatatgctttcacccagaaatttcactccttagcagtaaataaagaaatagtaactcttgttcatatacaccaaaggagaaatatacaggaatgtgcaaggcagaattataggtaatagcaaaaacaaaaactgaaaataacccagatgtctatcaacagtggaatggtaagtgaactgtttcatcaataaaggatgaataggagacattgaatacttttaagttgggtgaagcctacatgagtgtttgcttatttttgcaggtatcgtatacttaataaaaaacattaaaaaaatacatatgcattgtacaaaatttagactatctagaaatatacatatacgaaagtaaaattactcaagattcctaccacccacagataaccattgttaatatttcgatgcatatattttcaaacttcaaactacatagtgtgtatgttgtatatgtttgttttcactaatacatgtgaatatttttccttgtcatcaaatctacctaaatactttaaaaagaaaagatatggccgggcgcagtggctcatgcctgtaatcccaacacttcgggaggccgagg

SEQ ID NO: 19144 - RNA, 1616 nt, Homo sapiens
  source 1..1616: mol_type = other RNA
tgtaggcatgaggcagggcccaggcgcctccaggcgaaggcctccgctcccaccgctgcgagaggaggcgcgtccacgacggaataagcaggcggtcaggtcgccaacaatccggtcaaccacggtgcttcttccctggtgggtgtctggccccgttcttgctggggatggcgctcggggatgccaccgtgtttccccagggcccactgtgcaccctgcatgtcgcgcccttgtcacgggagcggcctgctgacccggagcacgcgtggccgtcacaaagggctgcaaagctgcagcaccagaacgcaaactcaggcgtgcggcaacggaggccacgttctcagccaccgtgccactctgcatgtcagctggctgggcgtgcctccgtcttgtgttagcaaggacatggcaatcacctgatttgctttggttgaagctccaggcagtacctggcccctcaccagactgaaaaagaaagtcccagaaccccagaaccccgtatggctcagaagtgccatcgagtactaggggtgcgccagggcccggctcagcccggccaagccccagcaggaaggaacatgtcctcaacgagaacatcctgcaaaatgcccggggtgggtgggggatgctcacggtgccagacgtgggctaggggccataaaggaccctcaggcaaggggcaaacacacccatgggtgtggccagctccctctacccatcaggacctccccagtggagggactgaaatgactcaggagcagatcaaggggcccagggcagaattctggagtcctacaaggcctgtgggaggctccccaaggggggctccaactttcaacctgagaagtctaagcctctatcaccatcatcatcgccatcgtcttcgccaccatcaggagttctggaagaagcgcccaagcatgggagacacagggatggttttgccagtgctgtgtgttaaggagctgctacctgctggggctgcttcagtaccctggagcaccatgagacacatctgtccccacgaggagctgaccactaggtcggggagctgagacatgggcaggtcacaccctgaattcgcatgcacgacacgacaagaggttccgactcgaggttcctggtttctaaggctcccaaacaataaacacaggtgccctcagcacagccgcccggctccttgttcagcagatgccacacagcccaaccttggtgtcctgaggcggccccactctaagcggggtggagcgacgaggctgcctggagacagagcagctccgtgggcccccagctcccctgccagattcccccacacaggcatggcccaagcaggcacctccgctcactcaggagtgctcagccctggtttggcctccctgtcagacagcctcaagccactaagccagcggcagccacagccaggacctcggaggctactgctttgttcttagagacagcaaaaccgcagagatgactcagaagacaaagagccccctccccggcctctcccaccatccagctgcctgaggggccgtcgcagtgcaggctctcccgagggccaggacgccctgtctgagcagggctccaggaacaatgaggctggccccggccacact

SEQ ID NO: 19145 - RNA, 2568 nt, Homo sapiens
  source 1..2568: mol_type = other RNA
tgtagtgtttcctactttatggatgaggaaactgaggcacagaaaaattaagtaacttgcccagagtcacataacagtaaatgctgtgatggtgtaattgaaacctgggcagtgggcgtcagactcatactccatagctcctggtgggttctgtctcttcctcctccctaccctctctctctctctctattggttttatcatacaggctttgtcccatttttggaagaggtggataccagcccctccttgcatcctacccattacgtttaatggcaaaaaccgcaatcacttttgcaccaaccaaatagaaagtaaagcttccattgtgtgcagatgaaatggtataattacttgaaaggaagagaggttcaaattgagaactggcactgatatctaatactgtcaaaatgaaacaggactatagagcaattactttaaagcaagagccatcgcttgtggaagacagctccctgtccagccggctttaaaagtatgaccctacacagcatttcctcattcagacacctactcagtttttaaagagtacatcagacaactgaactatccatgagtgctttactgaaaattcactttgatggcttaagtgagcactttggcattgtcccatgctaaaattattgaggccgcccatcactccatagacacaaggggccttgctcgcccaactcgattgaacccaaagcagatcctgaaggagactcttgtcctggcttcggggatccctgccccacacctcctggaaatcaataaaagtgacctcccacaggctcgacccatcatccgtgtcgctgggcagcaagagggcctggtcctgctgcaggctgcccacgcgttggcagcggtaggagtaaccagagggagcatatacgccagttgggttaaagactgcttggattgaattgttggaaatgatctcgactcggcgcaaactaaaccaactctggatggacaacttgttgtaattggtaaggatgaatcttatagcaagacttctggggtttccagcatcaccaagcttcaaagacaacctagcactttcttcactgcaatttgagttgtcagggtccacagttaccttctgaccaaatggctcgtctgtaaggtccagccaggtttgattcttaaatttaatcattattcttttggcccagaagagaatgcaaggaattccattgatggagacattaactgggccatgatggctgaatgcattccaaggttctttttctaaatgcccttctttgctcagattgtagttgagagcctgtgtgattggtattgttgtgaaattctggaatggtttcatatctccattattctgatcattcctcataaccacttctttatttgaagatgttggagaacttacattcttcctggcaaatatatggtccaaggttagtgaaagtcctataccttctctcctcaaacctttttctcccactctttctcttcactgatggccttgcatggcctacaggctccacatgttcctgtgtaactctcagaccccatctaatgccacactactcctcagtcactatgctccccttcttcactgatctttcagttcttagaaagcactagcccattctacatctgcacagagatgtcaccttaaactaccctatccagagtagccacccccatccccaagtcactatcacccatccagctatattttctctatagctctacagtatgtaaaaatcatctatttaattatttaatttacatctatctaactggtctgtcctctcacatttagaatataaactgtatcagagcagaaaccttcaccctcttaatttaaccgccatattcccggtacctacaacagcgtctggcacatagaaggcatttttaaacatccttgctgagtgaaccaatatcccagaaacctctcacagctagttcatcttacaggagaaacagtattaaagagttaattaaatggccaggcgcggtggctcacgcctgtaatcccagcacattgggaggccgaggcgggcggatcactcgaggtcaggagatcgacaccagcctggccaacatggtgaaaccccctctctactgaaaatacaaacatcagccaggcgtgatggtggaagcctgtaatcccagctactcaggaggctgaggtgggacaatcgcttgaacccgggaggcggaggttgtagtgagccaagatcgcaccactgcacaacagcctagaagacagagtgagaccctgtctcagaaaaaaataaaaataaaaataaataaatctataagtaaatgactcgccagtcaaaataaacggcaactttagggttaaaggcccaatctggctccaaagcttggggttttagttactacactacattgcttcactatattttacaatttactagctgcttataagtatgaattaaggctcagaagtctaattttccagactactcggaggactctcgccccactccactccacaaagattcagctcagcgactccttcctactctgacctagccccgcgtcccgctctcagtggcttgggcaagagc

SEQ ID NO: 19146 - RNA, 997 nt, Homo sapiens
  source 1..997: mol_type = other RNA
tgtcacccgctccttgcccagctccgggctccgtggcgacggcccctctcccgcgacggccgcctcccgtccgtcgccgccgtctcgggccctccccgccgacggaggttgccccgggctccttagcgccgaccgcggagccgcctcgccctcctgggcctctcgcggcggcagctcgggaccgtcggccggctgctcccagctcgctcggactgcggcctgggcctcgccgtcgtcgtcggactgcggccgccggggcgccttcttcgtccacacctccccctcctctgggccttgaagccgcgcgggcggcggccccctctctccgtccgacgccccggacctctgctcgcccgccgcgggcccgggcccctccaggaaggcggtgagacggcgcaaggccaggggcgagtacacggcgacggtgcgcgggaagcgcatgggccgcggggcgccgttctgggggctgccctgctccaggcctcgacgggatggctgctgggagaaagagccgccacccgtggtgccctcggccccggggccggccggggactcggggtcgcgggcccggcgctgcagcgtgcgcctccccagcgagcactgtaccgcggcgtcgatgcgcgggctcacctgcaccgccacgtcgcagctgccggccctgcgggcgcgcggcccgagacccggccccacctgcgccaggagagccatgagccgctcccgctggtagctgtcgaagtactcggcggccgtcagccgcccgcagcccgggaaggacaacgaggccgcgcccgccgagcagggggaggaggcgggaaggcagcccctgccgcgctgctgccagctgccgcccgccgcgcccttgcccttggtggccgcggggtatgggtaccggtacgagcagggggggcacgccgggaacacgtaaccgtccagcacctcgtcccccagggccgccatgggcgcactgctcccgcccgccgccgcaccctaaataggc

SEQ ID NO: 19147 - RNA, 921 nt, Homo sapiens
  source 1..921: mol_type = other RNA
tgtcctctgttcctcaggtctctgcttcattggtgtctccgggagactttctctcaccccaaccactctcagtaacagagaaatcctcaccatgcactcctgctttttgttattggggcaaaattctcacaaccgcacaggacgctctgattgacgcactgccaggagtagcgctctgtcttggggctgcagccggcctcctcagctcgagtgtaacaacagtcgtggccatggcagcaccagtcaatggcatcgcggggctggccatggcctcccaagccacaaaagcaaccatatttcatataggcgatgggggttcggggaccaacacaacccacagttcctgccagttccaggatcccacgccggtgcacacgtaatatcctggaggcctcgccggacccggggccaggtagaagcagcagcagcagcagcgacggcagtagcaggagcagcatgattggcaggcacacaggtagcggccccatcggagggtggcagaggtgggacggtgctgcagggccaccggaggcaccaagcccggcggacacacaccccggctgtcacgccccggctccgcccccgacctcaccttccctcgcggcccaagcagagccagctaggggcgggcacctggggcggcgcaaaggcgtcctgatctctgtatcttggtcactgaaggggctccagaggccgcggggcgctggggacaggaccgggagtcaggcccagggaagtctcctcggaataagggaggaaaaggcgctcttttgatgttattactcccccagcccctcccccgctcacctgggcgcccaaagggaacagaagacttggaggaggggtagtcctgaatttgctttaacattttattttatttggccgggcgcggtgactcacgcctgtaatcccagcactttg

SEQ ID NO: 19148 - RNA, 535 nt, Homo sapiens
  source 1..535: mol_type = other RNA
tgtctactactggagacactggagcagatccgacttagcaatggtgtttgcttcctccttatacgcagcgagctcagtggaggaacttgactggccaacatgctgggcgcgaaaacagcagaaaagggccttgaagatgttacgtccacgaggcttcttaggagaggacttggagaccaggccttgcttggtgagcaccagggcgtcttccctccgcgcctgggtgatgatggagccgtgttccatctaacaatcccgcgggcccgggctggctgggcgggaggacgggcgggcgcgcgggctgggctgggctggggggcctgggcgggggcccgctccggctcccgagactccgacttccacagctgttcacatcccccctctcgtttcctccccggaccgggaagggaggcggcctgtacaaagggcgggcggcccgggcagcggctcccccgggtgcccccggccccgatcccccagcggcagctccgggctcctcagtttgggtccaacatggagaatccggagcgaaaac

SEQ ID NO: 19149 - RNA, 540 nt, Homo sapiens
  source 1..540: mol_type = other RNA
tgtctactactggagacactggagcagatccgacttagcaatggtgtttgcttcctccttatacgcagcgagctcagtggaggaacttgactggccaacatgctgggcgcgaaaacagcagaaaagggccttgaagatgttacgtccacgaggcttcttaggagaggacttggagaccaggccttgcttggtgagcaccagggcgtcttccctccgcgcctgggtgatgatggagccgtgttccatctaacaatcccgcgggcccgggctggctgggcgggaggacgggcgggcgcgcgggctgggctgggctggggggcctgggcgggggcccgctccggctcccgagactccgacttccacagctgttcacatcccccctctcgtttcctccccggaccgggaagggaggcggcctgtacaaagggcgggcggcccgggcagcggctcccccgggtgcccccggccccgatcccccagcggcagctccgggctcctcagtttgggtccaacatggagaatccggagcgaaaacaagag

SEQ ID NO: 19150 - RNA, 8204 nt, Homo sapiens
  source 1..8204: mol_type = other RNA
tgtctatactctgtcactttaccagctgtttgatcttgggcaaactgacttgagacatttttgtattcgtaaaatggagctaatacttgcaattttgtcaagtcatcccagggattaagattacatatgcaaagatattggcacatagtaggagcacagtaagtatagctacataataatgctattaaacagagaaaaataaaagctgatacattttgaatcagaacagatgaggattagaaacgaagggatagaaatgaggaacatttttgaagaaaatgaccacctatacaaaatattattgttcaaatgtgaaaagcacaacataccattaaatttagtttgaaggaaatttatcctctcttatgttgatagtccttcagataaacagaactgatatttaatgatcggcatcagatggtaaatggtggtagggagctggagaaaaaacctgtgctgcaaaatcttcaaatgttgttggttctaagtggtgctggacaattgtttgcaggtatcgtgctctctcctcatagaagttttgatacaatggaatcagagatttcagagcacggcttgcatttatagctgttgctctaaccataatgggtagaacctttccattcacaatagcaccatcaaaaaggggaccaaagaagggaacctctggttttttcattatctgaatactgaacatgtgatttttcattggatatattacaataaggacatcaccaaattctgtgggaataattcctctcctgtagtctctagtatgctctgaccaaacaatgtgcacttcatcatttcccaaatgtctcaattttttggtcaaagaatcatcagaatcagaaggcattcttgttgacacgtgaaatattacctctactgtagaggtagcaaaatatggagtggtcaatccagtgcttttgtttttttgtagtcctcccataaaaccacaatggtttgtaagatttacctcccaaccaagaccagctacaaaatcttcatatgcttgacttcctcctgtattggtgagaatggagtgtttgtcttcttgtccttcagcaacataaaatactgcaatcttgtgtgtctctcggcactgccttgaatccaagttcctaagttctctaagtagcttttcatttttcttcaggagatgaaagctcctccgtttgtcccaggaattcattcccaatatactaagaagcaatctgcaataataaaatgctgactgaggtttttgaggtattggttcatcttgttccacagctttcatgtttaagtcattaaagtgcttctcaacaaattctttttcttctgtatgttgcttaaggatagcattaataacatcattttcttgtttttcagaaatgcacacaggttgtggagcaggaatattaagtgagattccagttctctgtaagcattcaggactagtaacacccaaatactgcaagagctcatcaagaacatcttcttcatctcttattgtatcccaagttggtacagtttctctaaatcttttaaactggagagaaagtccatcttttacggttatatcttctaagcattcattagatgtcggaggctcttctggcttctcttggtgagacaatgaaagcatgaaagatgtaggttctgacaagccacttacaggaggtgggccatacagtatagcagaatcccatgaatattttccagagagatcacgtactatgattctgacatttgaattggctgatgcaaggccagcagataaacctcctccaggcatattctcttctgatctgatctggatacaggacactaaggttgtattatttaacacaaagaactggatatttggactctcaaagagttcaggagaaagttcagtactttcactgtaatgattgtcgtgattttcacacacctgacttgttagcatagcaggaccaccgctcattggataatggcccaggtgatttaccagatgtgtaataacagtgcgggctgctatagagattaatccatgctgcatttgagttttcacttctgttactggctggagtttagaagatcgttctgagtcaggagagtgcagaggctcaggctctttcagactttccaaatgcataaaaggatcataatctacagatgccaaatcagagaggctcatgggaaaataccttggattgctaaaacactgagctccataaacacacccatgtaaaaccttataaatgcaattgagaacagatttttctgttttatcgctttctgctcccgtagcatgaaatggttggagcagtgtctttagaggtaaggccatgatccagtccagaaggcagagaagtaaagatactaccaacctcttgtccatttcataagatgaagcctctgtacttggtaaaagatgggtgatggtagctattaggatttgaataattttcaagggagaatcaggctggtaaatctgaagtctaggtacataatgaaccagcatgtgaagcatgttacaagctacgtgggctactgttttattagtaaactttaaggaaacacaaatcacattcagagcttccttaatttgaggatgatgagactcatggactagttcttcacaaatccaaatacctaaactacaaagtgctacacatcgtgcaggaccagagggctcatctcttgccgagcttaatacagttttgattataagttccttaacatctgtaaactgagacacagcaacatcaggaatgttgggatgaagagaaggcagttcacaatataagttgggaaagcaaaccaaagatcccagaagaacttgtgcttctactcttggtgcattgagaaaagctgaagaagccactctaccagctgctacaataaaatccataataagcattgtggcaccaggcaaaccaagtgaaaaaaattgaggtgagcagtgtttgatgattgtattgacaatatcctggtcaatatgaagtaatccacaatgcattatattgtagaaatgtgttagaaaatctctatttggagaaacatcttgtcttcttttcattgtattacaaataagtttatatgcatgtaatttaccttgtttatatttatcagtcaacatggttgccttaaaaagccaaggtgtaagaattctcagtggaggaattaaaactggtggagaaggggaggtcaggttatcagttgaaatgccaaggttatctctaatcttagctagattctgccaaagttcacagaggtaatcaaaaacttgagcatgtatttcaggatccatgattgaatttacatctcccaaaatgcctagcattcttcgccacattacagtagcaacatcagcatgccatccagtcagagtacctcctgccatcacactacaacattctgatggaaattcactaatttctagatcatctggtgtctgaagaacagagtggtggagcttctcgtcgagctgcagatccttctgttccatgtgatctatattcaatgtagaaggggaaggagtctgtgacctggagcccagaggtgagtggactggggaagcactttctgaaccagtaatagttgcaacttcagcagagaaagcttgctgattaagactgcttgtttcagaatctatatgaagagtagttagactagccacttcctgctcttcagcactctgatgatggccagaacctgaatccacatcagcagaggacgtaaccccagtgtcggttccaaagccaaaattgtcaaattttcggccatcatattggaaagcgctgaaagaatccgaatgactatctgagctgataagatcactgctccctgcactggcaggagaagtccattctgagggcacacctgggtcatcaatagggcgcatctggttctgcttgtttagaatatcagggaggtctttgggaatttccaggctgcctggactacttcctcttcttgtcatagtcgaggcattaccacttcgaagtcgttctgctataaactcatccatcagatcaggaacattagcactgctgccgccaatatcactattaagaggaggcagtttttggctcatgtcctctttattgactgcagctttccttccaaaatagcccattacatgactgtacagatccctcagtggagcctctggtggcattctgttctgcctctgtggggaaacatttgccttcggcttcgaaagagcatgtacaacagttttataaacgccacccagggagccctgctgtagtcctgcctcatgacttgatgacctaagagtactacgactacctaattgactacttgcaattccttctttttgtaatatggtggtgggaatctctgtggattccttcactgttttgctgcttactgatgcagtaccaagtgtatctagaggtctgtacacaccaggttttactagctctgtagcactatttgtgctggtatgggtgttgctagtgctgctattgctgctaccactactaaagccaccgagcttccgcagtctcatcttccatggagcctctttgttttccagaggattataaaactgaacggactcagtggatggcctaaaagtaacatgaacactatttcgttttttagtagcaattttcatgattttggctctatgagttactgtttcagacaagctccttttagttggagaaagtttgctagtacttgtaacatgaggcattctgcggttaacaggtgcttttagtgttgctttcttggcacgcataacatgtgggacagtgattttttcattaatttgcacactcttaagcttttcaactagtgttacatcaacacaagcatctaattctgtggctgcttgtctgtacagatgtttccttttttctttatcacaagggctatctaaactaggctctgatggctgtttatcagtgtttagttgcttagatttttcagaagtttgtgttctaaaaaaactgtctgactggttaggtgcgatattactcatgaagacagctgagtttggttctttctgaaactgtaggttttcaggagtcccaacaaaagaggtgatattttctgattcagtttcctgatctgtgcattctaatttatctaaggataatctttcacccctatttactgcaatagtcacttcctgagaagctgggtctttccctgtctcatttttactatgattttcctggttttccttaaaatattctttcagggtggaaagaagatcatcatctccttcaaggtcaatgtactggatttgttcaaaagctgaatctgcaagttctactggacctattaaatgacaaagatggtcatatatgctatcaccaacttccagagaagactctctactatgagtatcagtgatgtggctttcagtggatctagttattgaagaagcctctgtggaactctgcaagcttggtgcatgacgggatgaactgtcaatgacaggaactgcacctttggctcgttcaacagtgaatggttccaagatgtcagaagtgctgctacttcgaggcaatggctgctcctcattcaaagcaccaaaaacttcatttccagtttcttcactttgtgaaaaatgtctgactctagttgagcggggaagtatttgagcatcatcaatatctgaaagctcatcagaaaggggagtgagaacaatatcaggcaagaagggtttggaagtatggatcagaacaggagcacttttagcactgcgtatataggccgatggcagagcacattcaccaatggatcggcttctcatggcgacagttttttgccgtactatactcctcgccttttcggttcctggagaaccagtggttgttgcactcctctgtctcattggggcttggccaggctgatcacgactccatcctctagaaaatgacttgtcaactgaaactttctgaaattcatgtccaactcctttccctttgtgctttttttgtttctgttcactcagcttatccaatggtaaatcactgagatccaaactatataaattcctagctaaaactttagttaatgtctccatagtcagtgaccactcagtggccaactcttcccaataggtcagcgatgacaatactgacagtaagtcatcccaaagttctcgggagatgtacacatttaggtttgctttgatccaggcaactataagggtctggaaaagtggtcctgcaagtcgacctgccaaggtcatattttttttcccttggaactgtagaaaagcttgtgatggcatcttcagtacagattccgtgactctgagcaacacaagcagcatctgttcccaagtctttttgtccattgatacttgtacaaccatgtaccgataaatgttaagaatgcgtttacacatatctgtgtgttcatccagaagattttttatttcatttgcaggttcaagaagaaatatatttgatgagtttataataaacacctgcaaaactgcctgggtaccagctcgtatgttttgttctgtggcttcttcagaggcgttatgaagagcaccttggtaggagccgttttttgcccaactggaatttcgaacatgatcagcagtattggtcccattttcctcttctcttttttctccttcttccattgaaatatcatggtctgtgacattttcaatgcaagggaggtctgaagaagtgatcacaatttcttcaggctcttgcatgaacaaaggtttttcctcttgttggatccattcttgatatacttttaccacttttctcatagctgctgcttcacaaattggtaataaaaatgcctgacgaaatatctctgtcacaaagtttacattactccttttagaagaaaaaactctgcgaactatttcaatgtctgtgagatgttcttcatcaatactacagagactagatgagctaggttctcgctccgtgagagtgcttgtattggaatgagactgttcgggttctgtagttctgtctgttttatcagcattatcatttttgctttcttctctggatactaaactagcagctgctctctgaatattctttggcaagacttcaccttccatcccaggaatatgaggtcctgtatgtggttttggctccagccagaaagaaaccagccaacgaatgacaataacacgagccttaatgaaaggctcctttgtacaatagattgcttcattggtttcagcatctttctttatcacgacataatgtggctttggtctcatctgcgggatgtcaagtataggatgatataaactgttttccttacagatgtttggaaaaatataaggcaagtaatatttcttaaaatgtgaaaacaaaaatgaaaatcccctttcttggttttctttgttcttccattctaaactttttacctgaatgactatgtattttagaagtgcttcaagaaaatagcttgtgagatcttcttgccctttatctcctgattgtggggggacaagaggagtgatttcttctatagtgacttgagtttcttgaaggttgagtggaggattaatgagattatctaaagttcgaggtccatgttcagactgtggtgctgaaaatccagggattaagcatgaaaacatccagagctgttctttgctacagttattctgaagagcttgcaaccatagtaagaaaagacgaacaccttcccgcctaatctttaaggagtttcctgtgtgaagtagcttctttaaaatcaatccaatactatgaaactgccatcgctgatgaattctttctggaagaagttgtaaaattttctcaaaaataaaaagtatagcatccaattcctctctttgagacttgtgacctttctgtttaagactagcttcaatagtcacaaaattttcaaagaacacatagtatatatgtgaaaaatgttggtcgaaaaactgtttaagatcaatagattctgcattctcgatgacgatgcgcaggtgcttgaggcgagtcagtgcgtccttcttggtgtctagcaccttctgggtggacttcttcacgtccccgtgcggcttcttggagaacatcctgtcgctgccactgccactgccactgccacagccggctcccagccgggtcccggcggcagaaagtggagggagtggacggggaggagactagccagagaggctcattagctccccagccttgcgggccagggcagagccgactccttcccgatccaggccagggccgccacct

SEQ ID NO: 19151 - RNA, 2084 nt, Homo sapiens
  source 1..2084: mol_type = other RNA
tgtctctcgcccttggccttaggacccaacttctcttaccgccatggagttcgacctgggagcaggtgagctcctggggagtgtggactggaggtgcagggggccggactcaagcccagaagctgcctgcaccaaccacccaacttctctccacagccctggagcccacctcccagaagcccggtgtgggggcgggccacgggggagatcccaagctcagtccccacaaagttcagggccggtcggaggcaggggcaggtccgggtccaaaggtaagtcgcctcatcaccggctgcggaggggcgggaaggctggggttgcccctgaccccagggtcctgccttaggcctccaacttcagggggctgggtaaggggcgccgcctcactgccgcacctccatccagcaaggacaccacagctcttccgactccagcagcagctccagcgattcggacacggatgtgaaggtaaggggctctcgccagcgtccccaagcacgtgccctgcaccccagagaggcgtccccgcactggggctggcggggagggtgcggggagtggtccccctgtctcgcttccagcccagaaccatctcttctctcccatccctgccctcggccccacagtcccacgctgctggctccaagcagcacgagagcatcccgggcaaggccaagaagcccaaagtgaagaagaaggagaagggcaagaaggagaagggcaagaagaaggaggctccccactgaagggccctggacagggctcattaaaccttcctctctgccttctgcgactggtcagcgtggtgcctactctggcccgtccccagctccctgccccctgcccagcgctgggcccgcccattcgtgcgcgaggccaaggagaggctgtccacgccatgcccatcagggtttattgtttctgtaacagcggccacgccctggggcggtggcctgtgcagctggagatctctcagcaccttgggttgggggcggggctgggcgggacatgggatggaggcggtgcctgtggccagacagggtggaccttggggcctgcaggcaggagatgagttcggcggccacagtggcccccagcagcagcagcagcagcgggaggttcagcgggcgcgctcaccgcaccaggtggaaggtgagccagtacatgagcataggctgcgccgccgccaccgccatggtcaggtacatgcgcagctggttccgggccccacgcaccgggaccccctcagctgctgcgtctgccaagatcttcagccgcagcgtccggatcatgaacacaaagatggctacgcagcaccagcccagcaccaggtagtagccaatcttcccgaagagcaggcccatgaggaccccgccaatcatcccgacatatttgtagcccaagaaggccaccaggtcgatggtggtgaggtcggtgttgacagtgaccagatagaggctgagcaggatggccagcacctccagggtcagccaggccagggctgagctcgcttgcagccccaggaggtctggggagaacctatcctgggtccccagcgcaagaccagccaccaaaacgtaggtgatgaaagccattgctggaatgtagaggtccggggcattgacgtcaaagcggggggccaccggggtgtcctgttggtactgcacttcccagtcctggtgtaggtaggggaagaacagcaggcccagctttctgcccacatacatggtgtccacagcaaagtaatacttgagcttggtgatggggatgaagcggtcgatgttcttatccaccagctccttgccctgcgcggccaggctgctcccataggccatggccatgttggacaccgggtcagccaggaaggctgcatggggcgtgggagaggctgcaggataactcaggccaccaggtgcccgctgggccccatagccccggctctgggctgaacttgtgtcatcgaaaagctggtgggggtcggccatgcccggctgggacacagggatcctccgcttcgaggccgaacctggcatcccagcgctgtgcacacctcagggttccagatccttgatctcgtgacctct

SEQ ID NO: 19152 - RNA, 2054 nt, Homo sapiens
  source 1..2054: mol_type = other RNA
tgtctctcgcccttggccttaggacccaacttctcttaccgccatggagttcgacctgggagcaggtgagctcctggggagtgtggactggaggtgcagggggccggactcaagcccagaagctgcctgcaccaaccacccaacttctctccacagccctggagcccacctcccagaagcccggtgtgggggcgggccacgggggagatcccaagctcagtccccacaaagttcagggccggtcggaggcaggggcaggtccgggtccaaaggtaagtcgcctcatcaccggctgcggaggggcgggaaggctggggttgcccctgaccccagggtcctgccttaggcctccaacttcagggggctgggtaaggggcgccgcctcactgccgcacctccatccagcaaggacaccacagctcttccgactccagcagcagctccagcgattcggacacggatgtgaaggtaaggggctctcgccagcgtccccaagcacgtgccctgcaccccagagaggcgtccccgcactggggctggcggggagggtgcggggagtggtccccctgtctcgcttccagcccagaaccatctcttctctcccatccctgccctcggccccacagtcccacgctgctggctccaagcagcacgagagcatcccgggcaaggccaagaagcccaaagtgaagaagaaggagaagggcaagaaggagaagggcaagaagaaggaggctccccactgaagggccctggacagggctcattaaaccttcctctctgccttctgcgactggtcagcgtggtgcctactctggcccgtccccagctccctgccccctgcccagcgctgggcccgcccattcgtgcgcgaggccaaggagaggctgtccacgccatgcccatcagggtttattgtttctgtaacagcggccacgccctggggcggtggcctgtgcagctggagatctctcagcaccttgggttgggggcggggctgggcgggacatgggatggaggcggtgcctgtggccagacagggtggaccttggggcctgcaggcaggagatgagttcggcggccacagtggcccccagcagcagcagcagcagcgggaggttcagcgggcgcgctcaccgcaccaggtggaaggtgagccagtacatgagcataggctgcgccgccgccaccgccatggtcaggtacatgcgcagctggttccgggccccacgcaccgggaccccctcagctgctgcgtctgccaagatcttcagccgcagcgtccggatcatgaacacaaagatggctacgcagcaccagcccagcaccaggtagtagccaatcttcccgaagagcaggcccatgaggaccccgccaatcatcccgacatatttgtagcccaagaaggccaccaggtcgatggtggtgaggtcggtgttgacagtgaccagatagaggctgagcaggatggccagcacctccagggtcagccaggccagggctgagctcgcttgcagccccaggaggtctggggagaacctatcctgggtccccagcgcaagaccagccaccaaaacgtaggtgatgaaagccattgctggaatgtagaggtccggggcattgacgtcaaagcggggggccaccggggtgtcctgttggtactgcacttcccagtcctggtgtaggtaggggaagaacagcaggcccagctttctgcccacatacatggtgtccacagcaaagtaatacttgagcttggtgatggggatgaagcggtcgatgttcttatccaccagctccttgccctgcgcggccaggctgctcccataggccatggccatgttggacaccgggtcagccaggaaggctgcatggggcgtgggagaggctgcaggataactcaggccaccaggtgcccgctgggccccatagccccggctctgggctgaacttgtgtcatcgaaaagctggtgggggtcggccatgcccggctgggacacagggatcctccgcttcgaggctcagggttccagatccttgatctcgtgacctct

SEQ ID NO: 19153 - RNA, 2078 nt, Homo sapiens
  source 1..2078: mol_type = other RNA
tgtctctcgcccttggccttaggacccaacttctcttaccgccatggagttcgacctgggagcaggtgagctcctggggagtgtggactggaggtgcagggggccggactcaagcccagaagctgcctgcaccaaccacccaacttctctccacagccctggagcccacctcccagaagcccggtgtgggggcgggccacgggggagatcccaagctcagtccccacaaagttcagggccggtcggaggcaggggcaggtccgggtccaaaggtaagtcgcctcatcaccggctgcggaggggcgggaaggctggggttgcccctgaccccagggtcctgccttaggcctccaacttcagggggctgggtaaggggcgccgcctcactgccgcacctccatccagcaaggacaccacagctcttccgactccagcagcagctccagcgattcggacacggatgtgaaggtaaggggctctcgccagcgtccccaagcacgtgccctgcaccccagagaggcgtccccgcactggggctggcggggagggtgcggggagtggtccccctgtctcgcttccagcccagaaccatctcttctctcccatccctgccctcggccccacagtcccacgctgctggctccaagcagcacgagagcatcccgggcaaggccaagaagcccaaagtgaagaagaaggagaagggcaagaaggagaagggcaagaagaaggaggctccccactgaagggccctggacagggctcattaaaccttcctctctgccttctgcgactggtcagcgtggtgcctactctggcccgtccccagctccctgccccctgcccagcgctgggcccgcccattcgtgcgcgaggccaaggagaggctgtccacgccatgcccatcagggtttattgtttctgtaacagcggccacgccctggggcggtggcctgtgcagctggagatctctcagcaccttgggttgggggcggggctgggcgggacatgggatggaggcggtgcctgtggccagacagggtggaccttggggcctgcaggcaggagatgagttcggcggccacagtggcccccagcagcagcagcagcagcgggaggttcagcgggcgcgctcaccgcaccaggtggaaggtgagccagtacatgagcataggctgcgccgccgccaccgccatggtcaggtacatgcgcagctggttccgggccccacgcaccgggaccccctcagctgctgcgtctgccaagatcttcagccgcagcgtccggatcatgaacacaaagatggctacgcagcaccagcccagcaccaggtagtagccaatcttcccgaagagcaggcccatgaggaccccgccaatcatcccgacatatttgtagcccaagaaggccaccaggtcgatggtggtgaggtcggtgttgacagtgaccagatagaggctgagcaggatggccagcacctccagggtcagccaggccagggctgagctcgcttgcagccccaggaggtctggggagaacctatcctgggtccccagcgcaagaccagccaccaaaacgtaggtgatgaaagccattgctggaatgtagaggtccggggcattgacgtcaaagcggggggccaccggggtgtcctgttggtactgcacttcccagtcctggtgtaggtaggggaagaacagcaggcccagctttctgcccacatacatggtgtccacagcaaagtaatacttgagcttggtgatggggatgaagcggtcgatgttcttatccaccagctccttgccctgcgcggccaggctgctcccataggccatggccatgttggacaccgggtcagccaggaaggctgcatggggcgtgggagaggctgcaggataactcaggccaccaggtgcccgctgggccccatagccccggctctgggctgaacttgtgtcatcgaaaagctggtgggggtcggccatgcccggctgggacacagggatcctccgcttcgaggctggcatcccagcgctgtgcacacctcagggttccagatccttgatctcgtgacctct

SEQ ID NO: 19154 - RNA, 2099 nt, Homo sapiens
  source 1..2099: mol_type = other RNA
tgtctctcgcccttggccttaggacccaacttctcttaccgccatggagttcgacctgggagcaggtgagctcctggggagtgtggactggaggtgcagggggccggactcaagcccagaagctgcctgcaccaaccacccaacttctctccacagccctggagcccacctcccagaagcccggtgtgggggcgggccacgggggagatcccaagctcagtccccacaaagttcagggccggtcggaggcaggggcaggtccgggtccaaaggtaagtcgcctcatcaccggctgcggaggggcgggaaggctggggttgcccctgaccccagggtcctgccttaggcctccaacttcagggggctgggtaaggggcgccgcctcactgccgcacctccatccagcaaggacaccacagctcttccgactccagcagcagctccagcgattcggacacggatgtgaaggtaaggggctctcgccagcgtccccaagcacgtgccctgcaccccagagaggcgtccccgcactggggctggcggggagggtgcggggagtggtccccctgtctcgcttccagcccagaaccatctcttctctcccatccctgccctcggccccacagtcccacgctgctggctccaagcagcacgagagcatcccgggcaaggccaagaagcccaaagtgaagaagaaggagaagggcaagaaggagaagggcaagaagaaggaggctccccactgaagggccctggacagggctcattaaaccttcctctctgccttctgcgactggtcagcgtggtgcctactctggcccgtccccagctccctgccccctgcccagcgctgggcccgcccattcgtgcgcgaggccaaggagaggctgtccacgccatgcccatcagggtttattgtttctgtaacagcggccacgccctggggcggtggcctgtgcagctggagatctctcagcaccttgggttgggggcggggctgggcgggacatgggatggaggcggtgcctgtggccagacagggtggaccttggggcctgcaggcaggagatgagttcggcggccacagtggcccccagcagcagcagcagcagcgggaggttcagcgggcgcgctcaccgcaccaggtggaaggtgagccagtacatgagcataggctgcgccgccgccaccgccatggtcaggtacatgcgcagctggttccgggccccacgcaccgggaccccctcagctgctgcgtctgccaagatcttcagccgcagcgtccggatcatgaacacaaagatggctacgcagcaccagcccagcaccaggtagtagccaatcttcccgaagagcaggcccatgaggaccccgccaatcatcccgacatatttgtagcccaagaaggccaccaggtcgatggtggtgaggtcggtgttgacagtgaccagatagaggctgagcaggatggccagcacctccagggtcagccaggccagggctgagctcgcttgcagccccaggaggtctggggagaacctatcctgggtccccagcgcaagaccagccaccaaaacgtaggtgatgaaagccattgctggaatgtagaggtccggggcattgacgtcaaagcggggggccaccggggtgtcctgttggtactgcacttcccagtcctggtgtaggtaggggaagaacagcaggcccagctttctgcccacatacatggtgtccacagcaaagtaatacttgagcttggtgatggggatgaagcggtcgatgttcttatccaccagctccttgccctgcgcggccaggctgctcccataggccatggccatgttggacaccgggtcagccaggaaggctgcatggggcgtgggagaggctgcaggataactcaggccaccaggtgcccgctgggccccatagccccggctctgggctgaacttgtgtcatcgaaaagctggtgggggtcggccatgcccggctgggacacagggatcctccgcttcgagggcagccggggcgtccccgcagccgccgccgccaagcctgccgggtgcatccttcgccgccgccacctaagccgcggttc

SEQ ID NO: 19155 - RNA, 2108 nt, Homo sapiens
  source 1..2108: mol_type = other RNA
tgtctctcgcccttggccttaggacccaacttctcttaccgccatggagttcgacctgggagcaggtgagctcctggggagtgtggactggaggtgcagggggccggactcaagcccagaagctgcctgcaccaaccacccaacttctctccacagccctggagcccacctcccagaagcccggtgtgggggcgggccacgggggagatcccaagctcagtccccacaaagttcagggccggtcggaggcaggggcaggtccgggtccaaaggtaagtcgcctcatcaccggctgcggaggggcgggaaggctggggttgcccctgaccccagggtcctgccttaggcctccaacttcagggggctgggtaaggggcgccgcctcactgccgcacctccatccagcaaggacaccacagctcttccgactccagcagcagctccagcgattcggacacggatgtgaaggtaaggggctctcgccagcgtccccaagcacgtgccctgcaccccagagaggcgtccccgcactggggctggcggggagggtgcggggagtggtccccctgtctcgcttccagcccagaaccatctcttctctcccatccctgccctcggccccacagtcccacgctgctggctccaagcagcacgagagcatcccgggcaaggccaagaagcccaaagtgaagaagaaggagaagggcaagaaggagaagggcaagaagaaggaggctccccactgaagggccctggacagggctcattaaaccttcctctctgccttctgcgactggtcagcgtggtgcctactctggcccgtccccagctccctgccccctgcccagcgctgggcccgcccattcgtgcgcgaggccaaggagaggctgtccacgccatgcccatcagggtttattgtttctgtaacagcggccacgccctggggcggtggcctgtgcagctggagatctctcagcaccttgggttgggggcggggctgggcgggacatgggatggaggcggtgcctgtggccagacagggtggaccttggggcctgcaggcaggagatgagttcggcggccacagtggcccccagcagcagcagcagcagcgggaggttcagcgggcgcgctcaccgcaccaggtggaaggtgagccagtacatgagcataggctgcgccgccgccaccgccatggtcaggtacatgcgcagctggttccgggccccacgcaccgggaccccctcagctgctgcgtctgccaagatcttcagccgcagcgtccggatcatgaacacaaagatggctacgcagcaccagcccagcaccaggtagtagccaatcttcccgaagagcaggcccatgaggaccccgccaatcatcccgacatatttgtagcccaagaaggccaccaggtcgatggtggtgaggtcggtgttgacagtgaccagatagaggctgagcaggatggccagcacctccagggtcagccaggccagggctgagctcgcttgcagccccaggaggtctggggagaacctatcctgggtccccagcgcaagaccagccaccaaaacgtaggtgatgaaagccattgctggaatgtagaggtccggggcattgacgtcaaagcggggggccaccggggtgtcctgttggtactgcacttcccagtcctggtgtaggtaggggaagaacagcaggcccagctttctgcccacatacatggtgtccacagcaaagtaatacttgagcttggtgatggggatgaagcggtcgatgttcttatccaccagctccttgccctgcgcggccaggctgctcccataggccatggccatgttggacaccgggtcagccaggaaggctgcatggggcgtgggagaggctgcaggataactcaggccaccaggtgcccgctgggccccatagccccggctctgggctgaacttgtgtcatcgaaaagctggtgggggtcggccatgcccggctgggacacagggatcctccgcttcgagggccacttacgcagccggggcgtccccgcagccgccgccgccaagcctgccgggtgcatccttcgccgccgccacctaagccgcggttc

SEQ ID NO: 19156 - RNA, 2176 nt, Homo sapiens
  source 1..2176: mol_type = other RNA
tgtctctcgcccttggccttaggacccaacttctcttaccgccatggagttcgacctgggagcaggtgagctcctggggagtgtggactggaggtgcagggggccggactcaagcccagaagctgcctgcaccaaccacccaacttctctccacagccctggagcccacctcccagaagcccggtgtgggggcgggccacgggggagatcccaagctcagtccccacaaagttcagggccggtcggaggcaggggcaggtccgggtccaaaggtaagtcgcctcatcaccggctgcggaggggcgggaaggctggggttgcccctgaccccagggtcctgccttaggcctccaacttcagggggctgggtaaggggcgccgcctcactgccgcacctccatccagcaaggacaccacagctcttccgactccagcagcagctccagcgattcggacacggatgtgaaggtaaggggctctcgccagcgtccccaagcacgtgccctgcaccccagagaggcgtccccgcactggggctggcggggagggtgcggggagtggtccccctgtctcgcttccagcccagaaccatctcttctctcccatccctgccctcggccccacagtcccacgctgctggctccaagcagcacgagagcatcccgggcaaggccaagaagcccaaagtgaagaagaaggagaagggcaagaaggagaagggcaagaagaaggaggctccccactgaagggccctggacagggctcattaaaccttcctctctgccttctgcgactggtcagcgtggtgcctactctggcccgtccccagctccctgccccctgcccagcgctgggcccgcccattcgtgcgcgaggccaaggagaggctgtccacgccatgcccatcagggtttattgtttctgtaacagcggccacgccctggggcggtggcctgtgcagctggagatctctcagcaccttgggttgggggcggggctgggcgggacatgggatggaggcggtgcctgtggccagacagggtggaccttggggcctgcaggcaggagatgagttcggcggccacagtggcccccagcagcagcagcagcagcgggaggttcagcgggcgcgctcaccgcaccaggtggaaggtgagccagtacatgagcataggctgcgccgccgccaccgccatggtcaggtacatgcgcagctggttccgggccccacgcaccgggaccccctcagctgctgcgtctgccaagatcttcagccgcagcgtccggatctcgtgatccgaccgcctcggcctcccaaagtgctgggattacaagcatgagccaccgcgcccggcaaaaggggaaacatgaacacaaagatggctacgcagcaccagcccagcaccaggtagtagccaatcttcccgaagagcaggcccatgaggaccccgccaatcatcccgacatatttgtagcccaagaaggccaccaggtcgatggtggtgaggtcggtgttgacagtgaccagatagaggctgagcaggatggccagcacctccagggtcagccaggccagggctgagctcgcttgcagccccaggaggtctggggagaacctatcctgggtccccagcgcaagaccagccaccaaaacgtaggtgatgaaagccattgctggaatgtagaggtccggggcattgacgtcaaagcggggggccaccggggtgtcctgttggtactgcacttcccagtcctggtgtaggtaggggaagaacagcaggcccagctttctgcccacatacatggtgtccacagcaaagtaatacttgagcttggtgatggggatgaagcggtcgatgttcttatccaccagctccttgccctgcgcggccaggctgctcccataggccatggccatgttggacaccgggtcagccaggaaggctgcatggggcgtgggagaggctgcaggataactcaggccaccaggtgcccgctgggccccatagccccggctctgggctgaacttgtgtcatcgaaaagctggtgggggtcggccatgcccggctgggacacagggatcctccgcttcgagggcagccggggcgtccccgcagccgccgccgccaagcctgccgggtgcatccttcgccgccgccacctaagccgcggttc

SEQ ID NO: 19157 - RNA, 386 nt, Homo sapiens
  source 1..386: mol_type = other RNA
tgtcttactccctcaggcacatcctccagagataaaccacaggcacaggctcacacatggaaaataaagagacagaagacaagagtcagccatctagggtgcgggtatgctgtggacaacagagtgtgagcaacaggcaggaaatgttctgtgagcctccgcgagcgccaaccggctgtgagatgggcgagccactttgccagcgtggggctctctttcgggtcggttccctccccgccagcacacgcgcgaaccctcgcacctgggcacacacgcgcgcgcgtgcacacacacacacaaagttctgggggcccctctgcagaccggctcggctgcgctgggctcggagccgtgcgcccgccgggtccaggccggccctctcaccc

SEQ ID NO: 19158 - RNA, 301 nt, Homo sapiens
  source 1..301: mol_type = other RNA
tgtcttactccctcaggcacatcctccagagataaaccacaggcacaggctcacacatggaaaataaagagctccgcgagcgccaaccggctgtgagatgggcgagccactttgccagcgtggggctctctttcgggtcggttccctccccgccagcacacgcgcgaaccctcgcacctgggcacacacgcgcgcgcgtgcacacacacacacaaagttctgggggcccctctgcagaccggctcggctgcgctgggctcggagccgtgcgcccgccgggtccaggccggccctctcaccc

SEQ ID NO: 19159 - RNA, 37 nt, Homo sapiens
  source 1..37: mol_type = other RNA
tgtcttactccctcaggcacatctccaacaagtctct

SEQ ID NO: 19160 - RNA, 37 nt, Homo sapiens
  source 1..37: mol_type = other RNA
tgtcttactccctcaggcacatctccagcgagtctct

SEQ ID NO: 19161 - RNA, 1392 nt, Homo sapiens
  source 1..1392: mol_type = other RNA
tgtcttctctcctcccaaacagaagacggtcagtgcctctgaacctccctctgggctgggcacgcttggactcctccaaagagcttggaccagcctgagccacatccctgggcttgacttctccagaacaagcctcctggtctttctgggagagctctggcagcatcactgtgcctgtgcagggagagcgggaacccacttcctgcaccggctttctctgagttcttcaggatgaattcgctctggtctaggtaagttctaccccgaggccaccttcacttcccaaattccagcttttccttctctatccaaactgttacaaacacagtaacaataatttttaaaagctttttttttctctgaacacactaagtccctgctaattactgaaactccaggcattacaggaatatgtggacacttaaagaatcaggactacgtgggagagggggaggcagctccccagggtcctgggttggcacacaggctccaccactgtgtgactttcaacaagcgacttccttgaccagctgcccgctctgtaaaatggggagagtaatattcggccacactgagtcggtgtcaggttgagttaatatttggagagtttctggcacaggtaggtgctccttaagtgcctgttaaataagtgaagctttgagaaagtgtctaaaaggcgacacactaaatttttaagaggctggaggtgggccagggaggggaggtctcttatgtaatattttaatatctttttaaacctgaagaatgtgttcttgtagcactcctgtaattaaaacttaatgaactaaaagtacacccctcctgctcataccccttttgaactccgcagccgcgccccccagccggaggccccttgggcagcagacaatgggtgtggattcgccccaggtcccgccggctggggcggcgacaatacaccagtccccgacagctatttacatgacaagggcttccgggcgtgtctacgcgagttcccgtctttcctggtcgtcctccttgggttcgggtgaaagcgcttgggggttcagtgggccatgatccccgagctgctggagaactgaaggcggacagtctcctgcgaaaccaggcaatgggtgatccatcttgggggcttcctccccctttctccaatttctcttccctgagcccccagggaccttgtgctcctcagaagataggctagccccaagagcctgggtcaaggaccccagggacgggggcgaggggagggcgcaccagcaacccgcccgggtgcggctggcaccgagttcggctccccggccccgggcgtgcgccgggcaggcgttccaagctgaccgccgttggggagagggcacagcgcccctcctccgttgcgcgggtgccgggtct

SEQ ID NO: 19162 - RNA, 7581 nt, Homo sapiens
  source 1..7581: mol_type = other RNA
tgtcttctctcctcccaaacaggaacccgggtttcttgagctgccagtccctcaacccttggcagtgcttatttataccgtgaaattagcaccatcattacattttattgtgtgtgtgtacaaaacaatgatctattcttatttcaatttacactatagcagcctctggccctgttgcactggccctaggaagctcagctgagaactaactggccatagccaatgacaggctcccacagcaactaccaagcagtgacttggaatgtctacacatggaactgctcaaatgaaactcagcaagaaaggggctggaggcagctccttctctgccatgatctgagagaggttaggacactgggctcctctaacctggctgataaaccccaagaggatgacagtatcatttaaaaaaccttagtaaaatccaccttatagggactaagggtaaaacctatccaagtttcatgctgtcctcattactccctatgggggaatctgtcaggactaaactttctgccattctgttctcatgaggcaacattagaattacaacctgggagtccggctccagtgagcagacagtgccgagcctgggaagggatcaacagggtgtttcatgccctgaccatagtgtggggtgaaggatgtaaagaataaaataactattttcatcaatgctaaagatttggttcagaagagggtcaacacagtgatttaagtcatctcaaactcagtaacagggtaaagcagacatttaaaaatgaggatgtttctgtatcaatgacagctattttgctattagactgggttggctccagcaagataagcaaatgaggctttgaatgtaaatttcaacatttttcataatctttttctgacttagcagggctagatgtattggctttctagctacccatggagaatttcaacttttgccttgtccctggaaaaggcctcctggggagctggctccaaggcaaacactcttgagatctcaatttccaagcacatacccaaataccaccctgcgttaaggaccagaagttttctaagatgaaagatttccttttcactccaattcacatccctttggaaaaggggtcttattacaaacttcaggggacgtcccacagggctggcaaggccactccctccccaccttcctccaagagtcacatttcccaacagttgttgtgactctgcttctaattggatagtgactgctttcatgattttaaccatctagtatcacatgctgctactggtgggcccaatagctcaaatttctagtttccagtggttttctagttcccattcaatggcccttgaaggaagcccagatgtccatccattcagatgaagaactgctccccaaaatggctcagaagctgttttcccaggcaggtctggaacgaagcctccaatgaatggcggagaatggaaagaaccaaaataaaaccacaaagcagccaatcatggcccctttccctcactccctcctgtcctgtgagacatctagactgctgtcaagttgattacctaccaaagcctactttagagaagctactttagaatcaaacttctccacggaaaatttttacatggcctgcacgccctccccccgccccccccaaattcacagtttatttcatgaaacaaagagctacggtaatttaacacacaacatagtgaaaggagactctgacagtgcagtgcagatacctttttctgatcacaactacagatgactggagagaaaagggcacaggactggcaccaagcaaaccctactcatatgacctaaaagattagggaaagggacctactagctgcagttatatatttattattctcacacatgataaatacttaatataatgaactttaatgttctcggtgaatttctttaaaaatatctttttcatggtttaaaattcttttaaaagaaaataagatgctttacgttttctcttccttttgaacaaagagcttttcctctttgatgatgtgggaagagagagaggatgaaaggggagaactaggcaggtggaattcacagaggagattccgaggtctcagtgaaatgcagggataggcccctaaactcaggacagccctgcccagcctcgtccctctgcctgagttcaagtgtctcaacctcagagacagactttgggaaataaaagcagattctatttttaatctttagataaagcgcaaatgcttctataataactactgttccctccgtggaattgatgggagtaacctcaataagaacttgaggaaattgggaccaaatacagaatcctattgagagcgtgaaagccataactaagagataatggccaggagacgttagggccggggatggcctgctggctaagttggcaaagcagagaggtaaacatgttggtctaaggacaaaggaggggtagacaagtgggaggaaactagccaaacagcacttcctgttggcagtctgtgagctgggtgaatggtagggcagggtagcaccaacagatttcccagcccttgggccccagctcagggcagcagtaacagataatcagcagttaataggagtcatctcttagcctggacgttgctctaaacaccacctcttgccagtcttcagggaagggttctggcttgcctttgagctaagtcagcaggcaggtgctctcaatacagagcacagcaattctcagggaggcgaagaagaggactccctccactcaggagggaaaaggaatggggaaaagaaatttcccatcaggatctggtactcttcctgaagctggtgtgtctagctcagagcttgccagagattccctatgtccactgcccgaggctctgaaatctgaaagcacctgagtgttttagggaaatagggatggggtggattcatgtacaaagagaaaaataggtagaaacaaaagcaaagaaagagaagcttgccaaatgccttcttccactgctggaaatctacattcgcacagagcccgactgcccctgaccacctgctcctccaaggactgatcttgagactctgcacagcccagacaaaagcagcagcggcgaccccacagccaacagccttgctggcctcaatgcagcacccttgcatctatagaggagacctctgtgagtgtgcgcgcatgcacacgcacccatgcacaccgcagccaagagacacttcctcaacacaaccacttctggtgccacaaaggacatttcaaaatgagtctaaagccccagggcccctcagaacttcctgttacttcctggtcaaaggttcctgaaagccttggaatccaggctcacagggatgaggcctgtatctctcatcagtgactagcacccggcctagaacacgtgaatgctcaggaaatcgccactgatttgaaagaacaccatttcctcccaagggttcctaggtgccctcaatggggctctgtctggttggggaaatcgctttgagagcccctataccttccaacctgaccagcggaattgaattccatacttgactccagagtggactttttatttcacgatgaccatgtggaaaagttgggggaaagagacccaagtctgtctgtctccttggttggggcccactggattttcatacatggttcacacaaccataagcccccactggctaatgtcacaagagttctgagtgttgggatatgaggaaagaataacagtgggaaagtgttcggggcagatgtgtttttttttaagggggaaagaaagaaaagatttcccctccccaaatggtaccctgggggcagcttgtttgttcatgtgacattgattggtactacttctgttctgattctgcacacttgtgactggaaggagcctggttaagagctggaagtgtattttgctctggtttggggtcttgccctcttccaagagaccagcaagtctgtgccaatgtctgtgtgctcccagcagaccagcaagactgtgccagtgtctgtccagccactatgggccagagccctgcccgtgatgaggcttttcccagggcccagggactttgctctgtggttaccaacttcttttcttcagtggggagggaggctggggccttcccgagagacctaaaagattgcccactcttggcggcaagtgcaggtagttgctggcctccgaccatctgcttcgcctgcttcaccaggcccggggattggctaagaggccctggggtctgctcagcccctgcagaagctcttcctgaggcctgagttgttggctcatataaaaaggccttggcaggaggctgagaaagaagtctggcctgggtgagtgatttaacagcttgccaggggtcctctgaaggggctgctgctttcccagatgtctgaagaggatctgacacacagcctttctcaacagctctcggcatatgccccagacctttgctggcaggccatgaacttgactccaacactggcatcttctcatcagcctgtggtgtgacctgatgaggtgaagctgcccgctccttctggcgaggagttaggtctatgagatccatcaccaaagcagctctattttttgactgagtattctggtccacaggcctcagtgctttttctttagctacaagggtctggaccacagctgatagtactttctcaggaggtgggagtctctgggacaaagaggcatggggtttgtcagtaggcctgtctgaagtctggggtttgggactgctagtaatgagcagtctgtctggcggcggaagtctcaggccagtgggaactgaggttttctccagtgactggggccttgggctggcagcacctatggatttatccagccttgggtcagccgtccccagaggtctttccagtggttgggacctgactgagggtgaggagcttgggctggtcactggagagggtttgtcgcttagctggggtcttggtcctgccactgctggtggcctgtccagtggcctctggctggaaaccaaggattgggatttggtccctgacccagcgaggtctctgaccttatctaaaggctggggcctggagtcagttctctcaagaggtctttcaggtagcaatggcctctgacaagtccctgccagagcttttttggagagcgacagcatctggttggtgtcagcaggaggtttatctgacattttgggtgcctgagcagccattcctgttgattgctctgccaggtgagtgcttggccctggaggcagcggtactgggggaggcacatactcacggatctccccaggttccagaggattgggcccacaggggtcatgctcagtacaagacagacgcccatccagtttggaaatgaaaagcatcccttctcgatgctgcttacaaaaggagctggggcacatctcacagaaggaggctgcttccttcccgcagatgtcacactgatgccacggacattcccatttccctgctggtcgcttggtcagattgagacagtctgcgtggtaaacttttgggcagcctggtttcttgcaggagacgagctggccagcatccccacaactaaaacactcatcttctcgctcctttgtgatttcaccctgggtcctgcgctttccctgttgcttcttcttgaatttctttgacttttcttccgtggcaatgggttgattctttggccttacacccaagaagccactgcagttcggggctccacatttgcaaacagtctttccattcccaagacattctaggttgtagttgaaggtaagttcagtgcctgctttaatgtcacttagtgcaaaaaggcctacacgggtatctccattcacagaccacttctgtgtttcacagttgggctggcagcaatgattcatgaaccgagcatagtttcctttgggaccagcatcaatgattcggtctttgtctagggtgagcatatagaaattagtgatatcatgttcttgagcatagcgaattcgagctctgcattcttcttcatctataagctcacccacatactcattcacaaattcaccctttttaatatctgtttttgtccgtagaccccaaccccgctgtaatgtgcggaaaatttcaacctctggatattggcgcttggaaaagcactggttttgacagcgccctccggcaggacacactgtggggtggcactcatagagcagcatgcggttgatgcattcagagtctatcccacaggggttctcatcagtagctttacagttgcaacggggtatttcagataagtctgcagtgaagatctgtaccctgccaataggacggtttacctttatatgtttataaggtggtggcttcttgtcattctttcggtcttcctgcagctgtcttagctctttttgggcctttaattcctcaaaccttgctgcagcttcctgaagagcttttttatatgtcccatccactcctttgcccatcttatccttgctgctcacgtcaccctccatgtaagggaagactcgggcctggtgagtccacaaatagtcattagatccaaaaaagaggactgggaactctcccacatcatgtctcatcttatcaatgttggaaggaacagctcgaggatggcagatctcagctggccaccacctgtatcgtccaacttttacccagacaatctccctgtagtgtggctttttgcctgctttacagtcattgcaataccagtttccttcagggatatcaatgttcaggcattcacgatgaaaagcagcagggcaagaatcacagcacagaaggctgcctccttctgagcacacaaagcaccagctaacattaacatgctcatgatttcggcagccccgcctaggggtaaagtgattagggcagatgatactattagatgcaaggatctttgacccagcagccaggcaaaagtcattggcgtggtatgccacaggacagcggacacagcgcatcaaccgacctttagatgcagaaacattggctggattagcagcatgacaggttatacagatgtggagggagcaccggaagcccttgttctgcataacagtgggtgggtacttctggacacactcttcatggtaaaactttccacacaagggtagaaggcaccttttaacatcttccccactctgcttacatacaaaacaggtatggattcctgtgcgacattcattgcagataaattttcctcttggcatctcagtcaatccaaggcactccaggtggaaagccccacagcactgagcctcacataacagcagctcacccaatttttcacaattctgacagacattctccttgagtgcagctcctccaccgcgttcaccctgcatttttttagaggcaggcatcccgggatcgtgttctacaccttcctcaacagtctccttggggcttgtggccgtcctgtgaggcattagttctccagatgttcagccaatcactcgggcggactgcatgcaatgttagttctaaccctgctgtgattgggcgggtagtgggcgcctcatgccctgccactaactgctctgaggctgtttgttccactggaactttctgagctgttccattttaaggtttc

SEQ ID NO: 19163 - RNA, 11409 nt, Homo sapiens
  source 1..11409: mol_type = other RNA
tgtcttctctcctcccaaacaggaacccgggtttcttgagctgccagtccctcaacccttggcagtgcttatttataccgtgaaattagcaccatcattacattttattgtgtgtgtgtacaaaacaatgatctattcttatttcaatttacactatagcagcctctggccctgttgcactggccctaggaagctcagctgagaactaactggccatagccaatgacaggctcccacagcaactaccaagcagtgacttggaatgtctacacatggaactgctcaaatgaaactcagcaagaaaggggctggaggcagctccttctctgccatgatctgagagaggttaggacactgggctcctctaacctggctgataaaccccaagaggatgacagtatcatttaaaaaaccttagtaaaatccaccttatagggactaagggtaaaacctatccaagtttcatgctgtcctcattactccctatgggggaatctgtcaggactaaactttctgccattctgttctcatgaggcaacattagaattacaacctgggagtccggctccagtgagcagacagtgccgagcctgggaagggatcaacagggtgtttcatgccctgaccatagtgtggggtgaaggatgtaaagaataaaataactattttcatcaatgctaaagatttggttcagaagagggtcaacacagtgatttaagtcatctcaaactcagtaacagggtaaagcagacatttaaaaatgaggatgtttctgtatcaatgacagctattttgctattagactgggttggctccagcaagataagcaaatgaggctttgaatgtaaatttcaacatttttcataatctttttctgacttagcagggctagatgtattggctttctagctacccatggagaatttcaacttttgccttgtccctggaaaaggcctcctggggagctggctccaaggcaaacactcttgagatctcaatttccaagcacatacccaaataccaccctgcgttaaggaccagaagttttctaagatgaaagatttccttttcactccaattcacatccctttggaaaaggggtcttattacaaacttcaggggacgtcccacagggctggcaaggccactccctccccaccttcctccaagagtcacatttcccaacagttgttgtgactctgcttctaattggatagtgactgctttcatgattttaaccatctagtatcacatgctgctactggtgggcccaatagctcaaatttctagtttccagtggttttctagttcccattcaatggcccttgaaggaagcccagatgtccatccattcagatgaagaactgctccccaaaatggctcagaagctgttttcccaggcaggtctggaacgaagcctccaatgaatggcggagaatggaaagaaccaaaataaaaccacaaagcagccaatcatggcccctttccctcactccctcctgtcctgtgagacatctagactgctgtcaagttgattacctaccaaagcctactttagagaagctactttagaatcaaacttctccacggaaaatttttacatggcctgcacgccctccccccgccccccccaaattcacagtttatttcatgaaacaaagagctacggtaatttaacacacaacatagtgaaaggagactctgacagtgcagtgcagatacctttttctgatcacaactacagatgactggagagaaaagggcacaggactggcaccaagcaaaccctactcatatgacctaaaagattagggaaagggacctactagctgcagttatatatttattattctcacacatgataaatacttaatataatgaactttaatgttctcggtgaatttctttaaaaatatctttttcatggtttaaaattcttttaaaagaaaataagatgctttacgttttctcttccttttgaacaaagagcttttcctctttgatgatgtgggaagagagagaggatgaaaggggagaactaggcaggtggaattcacagaggagattccgaggtctcagtgaaatgcagggataggcccctaaactcaggacagccctgcccagcctcgtccctctgcctgagttcaagtgtctcaacctcagagacagactttgggaaataaaagcagattctatttttaatctttagataaagcgcaaatgcttctataataactactgttccctccgtggaattgatgggagtaacctcaataagaacttgaggaaattgggaccaaatacagaatcctattgagagcgtgaaagccataactaagagataatggccaggagacgttagggccggggatggcctgctggctaagttggcaaagcagagaggtaaacatgttggtctaaggacaaaggaggggtagacaagtgggaggaaactagccaaacagcacttcctgttggcagtctgtgagctgggtgaatggtagggcagggtagcaccaacagatttcccagcccttgggccccagctcagggcagcagtaacagataatcagcagttaataggagtcatctcttagcctggacgttgctctaaacaccacctcttgccagtcttcagggaagggttctggcttgcctttgagctaagtcagcaggcaggtgctctcaatacagagcacagcaattctcagggaggcgaagaagaggactccctccactcaggagggaaaaggaatggggaaaagaaatttcccatcaggatctggtactcttcctgaagctggtgtgtctagctcagagcttgccagagattccctatgtccactgcccgaggctctgaaatctgaaagcacctgagtgttttagggaaatagggatggggtggattcatgtacaaagagaaaaataggtagaaacaaaagcaaagaaagagaagcttgccaaatgccttcttccactgctggaaatctacattcgcacagagcccgactgcccctgaccacctgctcctccaaggactgatcttgagactctgcacagcccagacaaaagcagcagcggcgaccccacagccaacagccttgctggcctcaatgcagcacccttgcatctatagaggagacctctgtgagtgtgcgcgcatgcacacgcacccatgcacaccgcagccaagagacacttcctcaacacaaccacttctggtgccacaaaggacatttcaaaatgagtctaaagccccagggcccctcagaacttcctgttacttcctggtcaaaggttcctgaaagccttggaatccaggctcacagggatgaggcctgtatctctcatcagtgactagcacccggcctagaacacgtgaatgctcaggaaatcgccactgatttgaaagaacaccatttcctcccaagggttcctaggtgccctcaatggggctctgtctggttggggaaatcgctttgagagcccctataccttccaacctgaccagcggaattgaattccatacttgactccagagtggactttttatttcacgatgaccatgtggaaaagttgggggaaagagacccaagtctgtctgtctccttggttggggcccactggattttcatacatggttcacacaaccataagcccccactggctaatgtcacaagagttctgagtgttgggatatgaggaaagaataacagtgggaaagtgttcggggcagatgtgtttttttttaagggggaaagaaagaaaagatttcccctccccaaatggtaccctgggggcagcttgtttgttcatgtgacattgattggtactacttctgttctgattctgcacacttgtgactggaaggagcctggttaagagctggaagtgtattttgctctggtttggggtcttgccctcttccaagagaccagcaagtctgtgccaatgtctgtgtgctcccagcagaccagcaagactgtgccagtgtctgtccagccactatgggccagagccctgcccgtgatgaggcttttcccagggcccagggactttgctctgtggttaccaacttcttttcttcagtggggagggaggctggggccttcccgagagacctaaaagattgcccactcttggcggcaagtgcaggtagttgctggcctccgaccatctgcttcgcctgcttcaccaggcccggggattggctaagaggccctggggtctgctcagcccctgcagaagctcttcctgaggcctgagttgttggctcatataaaaaggccttggcaggaggctgagaaagaagtctggcctgggtgagtgatttaacagcttgccaggggtcctctgaaggggctgctgctttcccagatgtctgaagaggatctgacacacagcctttctcaacagctctcggcatatgccccagacctttgctggcaggccatgaacttgactccaacactggcatcttctcatcagcctgtggtgtgacctgatgaggtgaagctgcccgctccttctggcgaggagttaggtctatgagatccatcaccaaagcagctctattttttgactgagtattctggtccacaggcctcagtgctttttctttagctacaagggtctggaccacagctgatagtactttctcaggaggtgggagtctctgggacaaagaggcatggggtttgtcagtaggcctgtctgaagtctggggtttgggactgctagtaatgagcagtctgtctggcggcggaagtctcaggccagtgggaactgaggttttctccagtgactggggccttgggctggcagcacctatggatttatccagccttgggtcagccgtccccagaggtctttccagtggttgggacctgactgagggtgaggagcttgggctggtcactggagagggtttgtcgcttagctggggtcttggtcctgccactgctggtggcctgtccagtggcctctggctggaaaccaaggattgggatttggtccctgacccagcgaggtctctgaccttatctaaaggctggggcctggagtcagttctctcaagaggtctttcaggtagcaatggcctctgacaagtccctgccagagcttttttggagagcgacagcatctggttggtgtcagcaggaggtttatctgacattttgggtgcctgagcagccattcctgttgattgctctgccaggtgagtgcttggccctggaggcagcggtactgggggaggcacatactcacggatctccccaggttccagaggattgggcccacaggggtcatgctcagtacaagacagacgcccatccagtttggaaatgaaaagcatcccttctcgatgctgcttacaaaaggagctggggcacatctcacagaaggaggctgcttccttcccgcagatgtcacactgatgccacggacattcccatttccctgctggtcgcttggtcagattgagacagtctgcgtggtaaacttttgggcagcctggtttcttgcaggagacgagctggccagcatccccacaactaaaacactcatcttctcgctcctttgtgatttcaccctgggtcctgcgctttccctgttgcttcttcttgaatttctttgacttttcttccgtggcaatgggttgattctttggccttacacccaagaagccactgcagttcggggctccacatttgcaaacagtctttccattcccaagacattctaggttgtagttgaaggtaagttcagtgcctgctttaatgtcacttagtgcaaaaaggcctacacgggtatctccattcacagaccacttctgtgtttcacagttgggctggcagcaatgattcatgaaccgagcatagtttcctttgggaccagcatcaatgattcggtctttgtctagggtgagcatatagaaattagtgatatcatgttcttgagcatagcgaattcgagctctgcattcttcttcatctataagctcacccacatactcattcacaaattcaccctttttaatatctgtttttgtccgtagaccccaaccccgctgtaatgtgcggaaaatttcaacctctggatattggcgcttggaaaagcactggttttgacagcgccctccggcaggacacactgtggggtggcactcatagagcagcatgcggttgatgcattcagagtctatcccacaggggttctcatcagtagctttacagttgcaacggggtatttcagataagtctgcagtgaagatctgtaccctgccaataggacggtttacctttatatgtttataaggtggtggcttcttgtcattctttcggtcttcctgcagctgtcttagctctttttgggcctttaattcctcaaaccttgctgcagcttcctgaagagcttttttatatgtcccatccactcctttgcccatcttatccttgctgctcacgtcaccctccatgtaagggaagactcgggcctggtgagtccacaaatagtcattagatccaaaaaagaggactgggaactctcccacatcatgtctcatcttatcaatgttggaaggaacagctcgaggatggcagatctcagctggccaccacctgtatcgtccaacttttacccagacaatctccctgtagtgtggctttttgcctgctttacagtcattgcaataccagtttccttcagggatatcaatgttcaggcattcacgatgaaaagcagcagggcaagaatcacagcacagaaggctgcctccttctgagcacacaaagcaccagctaacattaacatgctcatgatttcggcagccccgcctaggggtaaagtgattagggcagatgatactattagatgcaaggatctttgacccagcagccaggcaaaagtcattggcgtggtatgccacaggacagcggacacagcgcatcaaccgacctttagatgcagaaacattggctggattagcagcatgacaggttatacagatgtggagggagcaccggaagcccttgttctgcataacagtgggtgggtacttctggacacactcttcatggtaaaactttccacacaagggtagaaggcaccttttaacatcttccccactctgcttacatacaaaacaggtatggattcctgtgcgacattcattgcagataaattttcctcttggcatctcagtcaatccaaggcactccaggtggaaagccccacagcactgagcctcacataacagcagctcacccaatttttcacaattctgacagacattctccttgagtgcagctcctccaccgcgttcaccctgcatttttttagaggcaggcatcccgggatcgtgttctacaccttcctcaacagtctccttggggcttgtggccgtcctgtgaggcattagttctccctctgagcctggaatctcttttgacgagtcatcatttttcacttttttacactgcatcttggctgcagcatgcctctgtcgttttcgcttccttggcttgtcaaatatcttggtagtgcctccaccaaaatcttttgaataagatgtggcacaagattcagttatgccattctccaggtgaccagcttcatagcactttttagaaaggccaaggtcccccttcttgggcataaatccagggtctaaatcattggattcaagaagtttcttagttggttttctttgacgtttactttcataatttcctggcgttttaactagcaattcctcagactcaagggcaggccgtggagagacttccggagccacaggcacagacaaggtcagctgcggcaactcagcatgtccacctccaagttctgactgagccaaggggccctccaaaaacggagcctccctttcaagaactggaggctcttctttggttgaaatcaaagaattctcgtccacctgcttgttctgagcactagatcgacctcgggctagaaggctttcctcttcacagcgggaacttaccttgtgcacctgctcctgtaccttcttttgttttttcttaggagcaaatatctgatcatattcttctgtatattccaaaagccacttgcttggcttcctaaggcgtttcttctctgaccgcacagctggttcagggagctcagcctgtggtgtcaaactgggaattcctggctccttttccatgtcaccaatgctggcactggatttatcacaaacatttaaccgtggcccagctgaatctaagcagtcagcatgattttgctctgtcagtggttcctcaagtatgcttgctgaaggagttctatgctctggaaactcatcccgcccctcctgcacagggtcactaggaagtaagaccctaaaggcacactcagagttttctttctctttaaatctgttcatgcgcttacgaggtttagtgcgcctttggtttaaacgctgccaccgctttttaggcaccacttgatttacaccattgagttcatcattctcactgttcattacagagtccagctctgggccttttccgttttcaaaagagagtcctttttcagaaattttaccaggatcagattgcttaaccttgctatcgaaatgcacatcagaaaaatggtcaccatcttcacttgttaagtggcccattatctgaaggggatcctctttactaggatcttctgccccacctctcaatgaacctccacgttctcggtctccctgcagtacagcatcaagagtcacacttggaagctgattcagttttcttttgcgctcggtctttaaggctttacggttcactgtgttctttaccatttgggctgaaaaagcatctcgcaatttggatgaaggctttgatcgtccacagttgcgcctagtaacacagtctgaacgacttttaccagaagcagggaggtctctcttgtcggacagtaagccaggtagggaagcagacaactcgccagataatgcagagtcacccccactagggctaggattggcggagttctgagtgccatctccctttttctctgaattgtgtgtggagcctcctgaaaccaaaaccttagagactcctacaggactattagtagaacagtccccacgaccaggactccggtaagagaccaggttttgagcagtcatcaaccgctgctccttcgtcttactatcatgcatatctttcaacatcattagcaatgtactgaatttgtagtctggttcaataggtatgtgattctgactagaagcagaagagaaaagtaatggttttgatggctttgatgttccagagtcactgacatcctcacctaaggatctgtaagagagttccttcaactcggataaaacatgtttcaccactgctgtttctatgtcacttgaatccctggttttctcatgcatattgttcagtagttttagaccatccactttcccacttttagaaatgctggccaaaggagagcctttggtatcagaagagcagcatttcaaactgcactcctcatttataactgggggttctgccataactggattttctttgtgtttgcactttatacttcggaacttgggctgtttgcttttcgaatgtaatagagcttgatttgctgccccaccctttattaacgagttctcactggatatgcttgatgacaggttgaattttggagagagagcatcatttgtaaaatctgactggggtttgtgaacaagagtagatgccttcagatcagagagattaacctgagacgtctcggttccaggctctgcactcttagtacaacccattaagtggtctgtatgtgagttactaatgagaggcttctgttttgcttttaccctagtgtttgtggcagcaaacctagaatactttatcttttcatttttctgcatagataacatgttctctgttctatcgaaagcatctggaatttcaaggacactgttatcagactctgagctgtgttctatgggatccaggtcactgcttccatcatcagaagtggtacagatactaatggaatcacttcgcttttcctcatcacctgctccaatatagcagagcttcacttttgaaccacacaccaggcttcgttggggtttattcttctctcgagaacactttgagatcaaagcaccctcaggcaagcccaataaagagtcaccatttgaagtctcaaattctttctttgcagtgttttttccacaggaagaaaacagaaaacttcctggggcagtgttggaccctgtgaggctatttgctatcctggaaagttcattagaggcctgcgtatcagatatatccccagagataaagtttaggccaaggttctctggaatctttcccctccgttcatctttatgtgcttcaaattgtatgtggccctttttcacactagtcctttttggattatcagagctctttctggctcgagatttagcgcaaggcttttccttctcatctgcagaatgttcagaatcaaaagccagtgatttcaaacagccattaagcaacaggtcatgttctgactcaggatcatttgtgcagtcttcaaatggcatatcttcttcactgtccaacttgattgaaccaggaatacattttcggttctttgaccccttgggaacatcatactgttctgcaagtccaacactggcttcccatttactcaaaattttctgaggaaccttatgcctatatcctttttctttctgtttccctcttctcctaaggacaggtagctcttcgaattgatgtctgccttcaaacatgacgattgcttttccagccacccaggctctctcagaaggatctccaaaagcctccacgtagtactgccgatagggcctccggttggaaactttcatttttgaatgtgtgttaatcaacggatcagaacaaatcctgcagggccaccatgggcgtctcttgaattttgcccagatgagatctccaacttcatacttcagtggcgtagactttttcttaggttgacaaaatggcaattcctgtgaagtagatgatgatgaagttccaggtaattctagcatgtttcctaatgtactggtactggaatctggatcatccgaaagggctgtccttgtcttcaggggcatctaaattcactggattggaaaagggcagcagacaatttcttctgggtagttcacaggtctgatccatcctgggccggcatcaaccgtgccccgcgccccctcccgggccagctggggggagggggtgaccctcattacactggggtgcgagcggagcggtggggagagagcggggccgctcgccgcacccccctccccccgcgtctctcttcaggggagaaggcagcgagcgcgacctgccccggcctattccgccgccgcctcctcctcctcacacccccaccgcgcgcgcc

SEQ ID NO: 19164 - RNA, 11300 nt, Homo sapiens
  source 1..11300: mol_type = other RNA
tgtcttctctcctcccaaacaggaacccgggtttcttgagctgccagtccctcaacccttggcagtgcttatttataccgtgaaattagcaccatcattacattttattgtgtgtgtgtacaaaacaatgatctattcttatttcaatttacactatagcagcctctggccctgttgcactggccctaggaagctcagctgagaactaactggccatagccaatgacaggctcccacagcaactaccaagcagtgacttggaatgtctacacatggaactgctcaaatgaaactcagcaagaaaggggctggaggcagctccttctctgccatgatctgagagaggttaggacactgggctcctctaacctggctgataaaccccaagaggatgacagtatcatttaaaaaaccttagtaaaatccaccttatagggactaagggtaaaacctatccaagtttcatgctgtcctcattactccctatgggggaatctgtcaggactaaactttctgccattctgttctcatgaggcaacattagaattacaacctgggagtccggctccagtgagcagacagtgccgagcctgggaagggatcaacagggtgtttcatgccctgaccatagtgtggggtgaaggatgtaaagaataaaataactattttcatcaatgctaaagatttggttcagaagagggtcaacacagtgatttaagtcatctcaaactcagtaacagggtaaagcagacatttaaaaatgaggatgtttctgtatcaatgacagctattttgctattagactgggttggctccagcaagataagcaaatgaggctttgaatgtaaatttcaacatttttcataatctttttctgacttagcagggctagatgtattggctttctagctacccatggagaatttcaacttttgccttgtccctggaaaaggcctcctggggagctggctccaaggcaaacactcttgagatctcaatttccaagcacatacccaaataccaccctgcgttaaggaccagaagttttctaagatgaaagatttccttttcactccaattcacatccctttggaaaaggggtcttattacaaacttcaggggacgtcccacagggctggcaaggccactccctccccaccttcctccaagagtcacatttcccaacagttgttgtgactctgcttctaattggatagtgactgctttcatgattttaaccatctagtatcacatgctgctactggtgggcccaatagctcaaatttctagtttccagtggttttctagttcccattcaatggcccttgaaggaagcccagatgtccatccattcagatgaagaactgctccccaaaatggctcagaagctgttttcccaggcaggtctggaacgaagcctccaatgaatggcggagaatggaaagaaccaaaataaaaccacaaagcagccaatcatggcccctttccctcactccctcctgtcctgtgagacatctagactgctgtcaagttgattacctaccaaagcctactttagagaagctactttagaatcaaacttctccacggaaaatttttacatggcctgcacgccctccccccgccccccccaaattcacagtttatttcatgaaacaaagagctacggtaatttaacacacaacatagtgaaaggagactctgacagtgcagtgcagatacctttttctgatcacaactacagatgactggagagaaaagggcacaggactggcaccaagcaaaccctactcatatgacctaaaagattagggaaagggacctactagctgcagttatatatttattattctcacacatgataaatacttaatataatgaactttaatgttctcggtgaatttctttaaaaatatctttttcatggtttaaaattcttttaaaagaaaataagatgctttacgttttctcttccttttgaacaaagagcttttcctctttgatgatgtgggaagagagagaggatgaaaggggagaactaggcaggtggaattcacagaggagattccgaggtctcagtgaaatgcagggataggcccctaaactcaggacagccctgcccagcctcgtccctctgcctgagttcaagtgtctcaacctcagagacagactttgggaaataaaagcagattctatttttaatctttagataaagcgcaaatgcttctataataactactgttccctccgtggaattgatgggagtaacctcaataagaacttgaggaaattgggaccaaatacagaatcctattgagagcgtgaaagccataactaagagataatggccaggagacgttagggccggggatggcctgctggctaagttggcaaagcagagaggtaaacatgttggtctaaggacaaaggaggggtagacaagtgggaggaaactagccaaacagcacttcctgttggcagtctgtgagctgggtgaatggtagggcagggtagcaccaacagatttcccagcccttgggccccagctcagggcagcagtaacagataatcagcagttaataggagtcatctcttagcctggacgttgctctaaacaccacctcttgccagtcttcagggaagggttctggcttgcctttgagctaagtcagcaggcaggtgctctcaatacagagcacagcaattctcagggaggcgaagaagaggactccctccactcaggagggaaaaggaatggggaaaagaaatttcccatcaggatctggtactcttcctgaagctggtgtgtctagctcagagcttgccagagattccctatgtccactgcccgaggctctgaaatctgaaagcacctgagtgttttagggaaatagggatggggtggattcatgtacaaagagaaaaataggtagaaacaaaagcaaagaaagagaagcttgccaaatgccttcttccactgctggaaatctacattcgcacagagcccgactgcccctgaccacctgctcctccaaggactgatcttgagactctgcacagcccagacaaaagcagcagcggcgaccccacagccaacagccttgctggcctcaatgcagcacccttgcatctatagaggagacctctgtgagtgtgcgcgcatgcacacgcacccatgcacaccgcagccaagagacacttcctcaacacaaccacttctggtgccacaaaggacatttcaaaatgagtctaaagccccagggcccctcagaacttcctgttacttcctggtcaaaggttcctgaaagccttggaatccaggctcacagggatgaggcctgtatctctcatcagtgactagcacccggcctagaacacgtgaatgctcaggaaatcgccactgatttgaaagaacaccatttcctcccaagggttcctaggtgccctcaatggggctctgtctggttggggaaatcgctttgagagcccctataccttccaacctgaccagcggaattgaattccatacttgactccagagtggactttttatttcacgatgaccatgtggaaaagttgggggaaagagacccaagtctgtctgtctccttggttggggcccactggattttcatacatggttcacacaaccataagcccccactggctaatgtcacaagagttctgagtgttgggatatgaggaaagaataacagtgggaaagtgttcggggcagatgtgtttttttttaagggggaaagaaagaaaagatttcccctccccaaatggtaccctgggggcagcttgtttgttcatgtgacattgattggtactacttctgttctgattctgcacacttgtgactggaaggagcctggttaagagctggaagtgtattttgctctggtttggggtcttgccctcttccaagagaccagcaagtctgtgccaatgtctgtgtgctcccagcagaccagcaagactgtgccagtgtctgtccagccactatgggccagagccctgcccgtgatgaggcttttcccagggcccagggactttgctctgtggttaccaacttcttttcttcagtggggagggaggctggggccttcccgagagacctaaaagattgcccactcttggcggcaagtgcaggtagttgctggcctccgaccatctgcttcgcctgcttcaccaggcccggggattggctaagaggccctggggtctgctcagcccctgcagaagctcttcctgaggcctgagttgttggctcatataaaaaggccttggcaggaggctgagaaagaagtctggcctgggtgagtgatttaacagcttgccaggggtcctctgaaggggctgctgctttcccagatgtctgaagaggatctgacacacagcctttctcaacagctctcggcatatgccccagacctttgctggcaggccatgaacttgactccaacactggcatcttctcatcagcctgtggtgtgacctgatgaggtgaagctgcccgctccttctggcgaggagttaggtctatgagatccatcaccaaagcagctctattttttgactgagtattctggtccacaggcctcagtgctttttctttagctacaagggtctggaccacagctgatagtactttctcaggaggtgggagtctctgggacaaagaggcatggggtttgtcagtaggcctgtctgaagtctggggtttgggactgctagtaatgagcagtctgtctggcggcggaagtctcaggccagtgggaactgaggttttctccagtgactggggccttgggctggcagcacctatggatttatccagccttgggtcagccgtccccagaggtctttccagtggttgggacctgactgagggtgaggagcttgggctggtcactggagagggtttgtcgcttagctggggtcttggtcctgccactgctggtggcctgtccagtggcctctggctggaaaccaaggattgggatttggtccctgacccagcgaggtctctgaccttatctaaaggctggggcctggagtcagttctctcaagaggtctttcaggtagcaatggcctctgacaagtccctgccagagcttttttggagagcgacagcatctggttggtgtcagcaggaggtttatctgacattttgggtgcctgagcagccattcctgttgattgctctgccaggtgagtgcttggccctggaggcagcggtactgggggaggcacatactcacggatctccccaggttccagaggattgggcccacaggggtcatgctcagtacaagacagacgcccatccagtttggaaatgaaaagcatcccttctcgatgctgcttacaaaaggagctggggcacatctcacagaaggaggctgcttccttcccgcagatgtcacactgatgccacggacattcccatttccctgctggtcgcttggtcagattgagacagtctgcgtggtaaacttttgggcagcctggtttcttgcaggagacgagctggccagcatccccacaactaaaacactcatcttctcgctcctttgtgatttcaccctgggtcctgcgctttccctgttgcttcttcttgaatttctttgacttttcttccgtggcaatgggttgattctttggccttacacccaagaagccactgcagttcggggctccacatttgcaaacagtctttccattcccaagacattctaggttgtagttgaaggtaagttcagtgcctgctttaatgtcacttagtgcaaaaaggcctacacgggtatctccattcacagaccacttctgtgtttcacagttgggctggcagcaatgattcatgaaccgagcatagtttcctttgggaccagcatcaatgattcggtctttgtctagggtgagcatatagaaattagtgatatcatgttcttgagcatagcgaattcgagctctgcattcttcttcatctataagctcacccacatactcattcacaaattcaccctttttaatatctgtttttgtccgtagaccccaaccccgctgtaatgtgcggaaaatttcaacctctggatattggcgcttggaaaagcactggttttgacagcgccctccggcaggacacactgtggggtggcactcatagagcagcatgcggttgatgcattcagagtctatcccacaggggttctcatcagtagctttacagttgcaacggggtatttcagataagtctgcagtgaagatctgtaccctgccaataggacggtttacctttatatgtttataaggtggtggcttcttgtcattctttcggtcttcctgcagctgtcttagctctttttgggcctttaattcctcaaaccttgctgcagcttcctgaagagcttttttatatgtcccatccactcctttgcccatcttatccttgctgctcacgtcaccctccatgtaagggaagactcgggcctggtgagtccacaaatagtcattagatccaaaaaagaggactgggaactctcccacatcatgtctcatcttatcaatgttggaaggaacagctcgaggatggcagatctcagctggccaccacctgtatcgtccaacttttacccagacaatctccctgtagtgtggctttttgcctgctttacagtcattgcaataccagtttccttcagggatatcaatgttcaggcattcacgatgaaaagcagcagggcaagaatcacagcacagaaggctgcctccttctgagcacacaaagcaccagctaacattaacatgctcatgatttcggcagccccgcctaggggtaaagtgattagggcagatgatactattagatgcaaggatctttgacccagcagccaggcaaaagtcattggcgtggtatgccacaggacagcggacacagcgcatcaaccgacctttagatgcagaaacattggctggattagcagcatgacaggttatacagatgtggagggagcaccggaagcccttgttctgcataacagtgggtgggtacttctggacacactcttcatggtaaaactttccacacaagggtagaaggcaccttttaacatcttccccactctgcttacatacaaaacaggtatggattcctgtgcgacattcattgcagataaattttcctcttggcatctcagtcaatccaaggcactccaggtggaaagccccacagcactgagcctcacataacagcagctcacccaatttttcacaattctgacagacattctccttgagtgcagctcctccaccgcgttcaccctgcatttttttagaggcaggcatcccgggatcgtgttctacaccttcctcaacagtctccttggggcttgtggccgtcctgtgaggcattagttctccctctgagcctggaatctcttttgacgagtcatcatttttcacttttttacactgcatcttggctgcagcatgcctctgtcgttttcgcttccttggcttgtcaaatatcttggtagtgcctccaccaaaatcttttgaataagatgtggcacaagattcagttatgccattctccaggtgaccagcttcatagcactttttagaaaggccaaggtcccccttcttgggcataaatccagggtctaaatcattggattcaagaagtttcttagttggttttctttgacgtttactttcataatttcctggcgttttaactagcaattcctcagactcaagggcaggccgtggagagacttccggagccacaggcacagacaaggtcagctgcggcaactcagcatgtccacctccaagttctgactgagccaaggggccctccaaaaacggagcctccctttcaagaactggaggctcttctttggttgaaatcaaagaattctcgtccacctgcttgttctgagcactagatcgacctcgggctagaaggctttcctcttcacagcgggaacttaccttgtgcacctgctcctgtaccttcttttgttttttcttaggagcaaatatctgatcatattcttctgtatattccaaaagccacttgcttggcttcctaaggcgtttcttctctgaccgcacagctggttcagggagctcagcctgtggtgtcaaactgggaattcctggctccttttccatgtcaccaatgctggcactggatttatcacaaacatttaaccgtggcccagctgaatctaagcagtcagcatgattttgctctgtcagtggttcctcaagtatgcttgctgaaggagttctatgctctggaaactcatcccgcccctcctgcacagggtcactaggaagtaagaccctaaaggcacactcagagttttctttctctttaaatctgttcatgcgcttacgaggtttagtgcgcctttggtttaaacgctgccaccgctttttaggcaccacttgatttacaccattgagttcatcattctcactgttcattacagagtccagctctgggccttttccgttttcaaaagagagtcctttttcagaaattttaccaggatcagattgcttaaccttgctatcgaaatgcacatcagaaaaatggtcaccatcttcacttgttaagtggcccattatctgaaggggatcctctttactaggatcttctgccccacctctcaatgaacctccacgttctcggtctccctgcagtacagcatcaagagtcacacttggaagctgattcagttttcttttgcgctcggtctttaaggctttacggttcactgtgttctttaccatttgggctgaaaaagcatctcgcaatttggatgaaggctttgatcgtccacagttgcgcctagtaacacagtctgaacgacttttaccagaagcagggaggtctctcttgtcggacagtaagccaggtagggaagcagacaactcgccagataatgcagagtcacccccactagggctaggattggcggagttctgagtgccatctccctttttctctgaattgtgtgtggagcctcctgaaaccaaaaccttagagactcctacaggactattagtagaacagtccccacgaccaggactccggtaagagaccaggttttgagcagtcatcaaccgctgctccttcgtcttactatcatgcatatctttcaacatcattagcaatgtactgaatttgtagtctggttcaataggtatgtgattctgactagaagcagaagagaaaagtaatggttttgatggctttgatgttccagagtcactgacatcctcacctaaggatctgtaagagagttccttcaactcggataaaacatgtttcaccactgctgtttctatgtcacttgaatccctggttttctcatgcatattgttcagtagttttagaccatccactttcccacttttagaaatgctggccaaaggagagcctttggtatcagaagagcagcatttcaaactgcactcctcatttataactgggggttctgccataactggattttctttgtgtttgcactttatacttcggaacttgggctgtttgcttttcgaatgtaatagagcttgatttgctgccccaccctttattaacgagttctcactggatatgcttgatgacaggttgaattttggagagagagcatcatttgtaaaatctgactggggtttgtgaacaagagtagatgccttcagatcagagagattaacctgagacgtctcggttccaggctctgcactcttagtacaacccattaagtggtctgtatgtgagttactaatgagaggcttctgttttgcttttaccctagtgtttgtggcagcaaacctagaatactttatcttttcatttttctgcatagataacatgttctctgttctatcgaaagcatctggaatttcaaggacactgttatcagactctgagctgtgttctatgggatccaggtcactgcttccatcatcagaagtggtacagatactaatggaatcacttcgcttttcctcatcacctgctccaatatagcagagcttcacttttgaaccacacaccaggcttcgttggggtttattcttctctcgagaacactttgagatcaaagcaccctcaggcaagcccaataaagagtcaccatttgaagtctcaaattctttctttgcagtgttttttccacaggaagaaaacagaaaacttcctggggcagtgttggaccctgtgaggctatttgctatcctggaaagttcattagaggcctgcgtatcagatatatccccagagataaagtttaggccaaggttctctggaatctttcccctccgttcatctttatgtgcttcaaattgtatgtggccctttttcacactagtcctttttggattatcagagctctttctggctcgagatttagcgcaaggcttttccttctcatctgcagaatgttcagaatcaaaagccagtgatttcaaacagccattaagcaacaggtcatgttctgactcaggatcatttgtgcagtcttcaaatggcatatcttcttcactgtccaacttgattgaaccaggaatacattttcggttctttgaccccttgggaacatcatactgttctgcaagtccaacactggcttcccatttactcaaaattttctgaggaaccttatgcctatatcctttttctttctgtttccctcttctcctaaggacaggtagctcttcgaattgatgtctgccttcaaacatgacgattgcttttccagccacccaggctctctcagaaggatctccaaaagcctccacgtagtactgccgatagggcctccggttggaaactttcatttttgaatgtgtgttaatcaacggatcagaacaaatcctgcagggccaccatgggcgtctcttgaattttgcccagatgagatctccaacttcatacttcagtggcgtagactttttcttaggttgacaaaatggcaattcctgtgaagtagatgatgatgaagttccaggtaattctagcatgtttcctaatgtactggtactggaatctggatcatccgaaagggctgtccttgtcttcaggggcatctaaattcactggattggaaaagggcagcagacaatttcttctgggtagttcacaggtctgatccatcctgggccggcatcaacctcaggagttacctggtccctagggcgctaagcgccttctcgctgttcagagaaagccggatccggccgccataaaaattccgcctcctccagaaagcct

SEQ ID NO: 19165 - RNA, 11217 nt, Homo sapiens
  source 1..11217: mol_type = other RNA
tgtcttctctcctcccaaacaggaacccgggtttcttgagctgccagtccctcaacccttggcagtgcttatttataccgtgaaattagcaccatcattacattttattgtgtgtgtgtacaaaacaatgatctattcttatttcaatttacactatagcagcctctggccctgttgcactggccctaggaagctcagctgagaactaactggccatagccaatgacaggctcccacagcaactaccaagcagtgacttggaatgtctacacatggaactgctcaaatgaaactcagcaagaaaggggctggaggcagctccttctctgccatgatctgagagaggttaggacactgggctcctctaacctggctgataaaccccaagaggatgacagtatcatttaaaaaaccttagtaaaatccaccttatagggactaagggtaaaacctatccaagtttcatgctgtcctcattactccctatgggggaatctgtcaggactaaactttctgccattctgttctcatgaggcaacattagaattacaacctgggagtccggctccagtgagcagacagtgccgagcctgggaagggatcaacagggtgtttcatgccctgaccatagtgtggggtgaaggatgtaaagaataaaataactattttcatcaatgctaaagatttggttcagaagagggtcaacacagtgatttaagtcatctcaaactcagtaacagggtaaagcagacatttaaaaatgaggatgtttctgtatcaatgacagctattttgctattagactgggttggctccagcaagataagcaaatgaggctttgaatgtaaatttcaacatttttcataatctttttctgacttagcagggctagatgtattggctttctagctacccatggagaatttcaacttttgccttgtccctggaaaaggcctcctggggagctggctccaaggcaaacactcttgagatctcaatttccaagcacatacccaaataccaccctgcgttaaggaccagaagttttctaagatgaaagatttccttttcactccaattcacatccctttggaaaaggggtcttattacaaacttcaggggacgtcccacagggctggcaaggccactccctccccaccttcctccaagagtcacatttcccaacagttgttgtgactctgcttctaattggatagtgactgctttcatgattttaaccatctagtatcacatgctgctactggtgggcccaatagctcaaatttctagtttccagtggttttctagttcccattcaatggcccttgaaggaagcccagatgtccatccattcagatgaagaactgctccccaaaatggctcagaagctgttttcccaggcaggtctggaacgaagcctccaatgaatggcggagaatggaaagaaccaaaataaaaccacaaagcagccaatcatggcccctttccctcactccctcctgtcctgtgagacatctagactgctgtcaagttgattacctaccaaagcctactttagagaagctactttagaatcaaacttctccacggaaaatttttacatggcctgcacgccctccccccgccccccccaaattcacagtttatttcatgaaacaaagagctacggtaatttaacacacaacatagtgaaaggagactctgacagtgcagtgcagatacctttttctgatcacaactacagatgactggagagaaaagggcacaggactggcaccaagcaaaccctactcatatgacctaaaagattagggaaagggacctactagctgcagttatatatttattattctcacacatgataaatacttaatataatgaactttaatgttctcggtgaatttctttaaaaatatctttttcatggtttaaaattcttttaaaagaaaataagatgctttacgttttctcttccttttgaacaaagagcttttcctctttgatgatgtgggaagagagagaggatgaaaggggagaactaggcaggtggaattcacagaggagattccgaggtctcagtgaaatgcagggataggcccctaaactcaggacagccctgcccagcctcgtccctctgcctgagttcaagtgtctcaacctcagagacagactttgggaaataaaagcagattctatttttaatctttagataaagcgcaaatgcttctataataactactgttccctccgtggaattgatgggagtaacctcaataagaacttgaggaaattgggaccaaatacagaatcctattgagagcgtgaaagccataactaagagataatggccaggagacgttagggccggggatggcctgctggctaagttggcaaagcagagaggtaaacatgttggtctaaggacaaaggaggggtagacaagtgggaggaaactagccaaacagcacttcctgttggcagtctgtgagctgggtgaatggtagggcagggtagcaccaacagatttcccagcccttgggccccagctcagggcagcagtaacagataatcagcagttaataggagtcatctcttagcctggacgttgctctaaacaccacctcttgccagtcttcagggaagggttctggcttgcctttgagctaagtcagcaggcaggtgctctcaatacagagcacagcaattctcagggaggcgaagaagaggactccctccactcaggagggaaaaggaatggggaaaagaaatttcccatcaggatctggtactcttcctgaagctggtgtgtctagctcagagcttgccagagattccctatgtccactgcccgaggctctgaaatctgaaagcacctgagtgttttagggaaatagggatggggtggattcatgtacaaagagaaaaataggtagaaacaaaagcaaagaaagagaagcttgccaaatgccttcttccactgctggaaatctacattcgcacagagcccgactgcccctgaccacctgctcctccaaggactgatcttgagactctgcacagcccagacaaaagcagcagcggcgaccccacagccaacagccttgctggcctcaatgcagcacccttgcatctatagaggagacctctgtgagtgtgcgcgcatgcacacgcacccatgcacaccgcagccaagagacacttcctcaacacaaccacttctggtgccacaaaggacatttcaaaatgagtctaaagccccagggcccctcagaacttcctgttacttcctggtcaaaggttcctgaaagccttggaatccaggctcacagggatgaggcctgtatctctcatcagtgactagcacccggcctagaacacgtgaatgctcaggaaatcgccactgatttgaaagaacaccatttcctcccaagggttcctaggtgccctcaatggggctctgtctggttggggaaatcgctttgagagcccctataccttccaacctgaccagcggaattgaattccatacttgactccagagtggactttttatttcacgatgaccatgtggaaaagttgggggaaagagacccaagtctgtctgtctccttggttggggcccactggattttcatacatggttcacacaaccataagcccccactggctaatgtcacaagagttctgagtgttgggatatgaggaaagaataacagtgggaaagtgttcggggcagatgtgtttttttttaagggggaaagaaagaaaagatttcccctccccaaatggtaccctgggggcagcttgtttgttcatgtgacattgattggtactacttctgttctgattctgcacacttgtgactggaaggagcctggttaagagctggaagtgtattttgctctggtttggggtcttgccctcttccaagagaccagcaagtctgtgccaatgtctgtgtgctcccagcagaccagcaagactgtgccagtgtctgtccagccactatgggccagagccctgcccgtgatgaggcttttcccagggcccagggactttgctctgtggttaccaacttcttttcttcagtggggagggaggctggggccttcccgagagacctaaaagattgcccactcttggcggcaagtgcaggtagttgctggcctccgaccatctgcttcgcctgcttcaccaggcccggggattggctaagaggccctggggtctgctcagcccctgcagaagctcttcctgaggcctgagttgttggctcatataaaaaggccttggcaggaggctgagaaagaagtctggcctgggtgagtgatttaacagcttgccaggggtcctctgaaggggctgctgctttcccagatgtctgaagaggatctgacacacagcctttctcaacagctctcggcatatgccccagacctttgctggcaggccatgaacttgactccaacactggcatcttctcatcagcctgtggtgtgacctgatgaggtgaagctgcccgctccttctggcgaggagttaggtctatgagatccatcaccaaagcagctctattttttgactgagtattctggtccacaggcctcagtgctttttctttagctacaagggtctggaccacagctgatagtactttctcaggaggtgggagtctctgggacaaagaggcatggggtttgtcagtaggcctgtctgaagtctggggtttgggactgctagtaatgagcagtctgtctggcggcggaagtctcaggccagtgggaactgaggttttctccagtgactggggccttgggctggcagcacctatggatttatccagccttgggtcagccgtccccagaggtctttccagtggttgggacctgactgagggtgaggagcttgggctggtcactggagagggtttgtcgcttagctggggtcttggtcctgccactgctggtggcctgtccagtggcctctggctggaaaccaaggattgggatttggtccctgacccagcgaggtctctgaccttatctaaaggctggggcctggagtcagttctctcaagaggtctttcaggtagcaatggcctctgacaagtccctgccagagcttttttggagagcgacagcatctggttggtgtcagcaggaggtttatctgacattttgggtgcctgagcagccattcctgttgattgctctgccaggtgagtgcttggccctggaggcagcggtactgggggaggcacatactcacggatctccccaggttccagaggattgggcccacaggggtcatgctcagtacaagacagacgcccatccagtttggaaatgaaaagcatcccttctcgatgctgcttacaaaaggagctggggcacatctcacagaaggaggctgcttccttcccgcagatgtcacactgatgccacggacattcccatttccctgctggtcgcttggtcagattgagacagtctgcgtggtaaacttttgggcagcctggtttcttgcaggagacgagctggccagcatccccacaactaaaacactcatcttctcgctcctttgtgatttcaccctgggtcctgcgctttccctgttgcttcttcttgaatttctttgacttttcttccgtggcaatgggttgattctttggccttacacccaagaagccactgcagttcggggctccacatttgcaaacagtctttccattcccaagacattctaggttgtagttgaaggtaagttcagtgcctgctttaatgtcacttagtgcaaaaaggcctacacgggtatctccattcacagaccacttctgtgtttcacagttgggctggcagcaatgattcatgaaccgagcatagtttcctttgggaccagcatcaatgattcggtctttgtctagggtgagcatatagaaattagtgatatcatgttcttgagcatagcgaattcgagctctgcattcttcttcatctataagctcacccacatactcattcacaaattcaccctttttaatatctgtttttgtccgtagaccccaaccccgctgtaatgtgcggaaaatttcaacctctggatattggcgcttggaaaagcactggttttgacagcgccctccggcaggacacactgtggggtggcactcatagagcagcatgcggttgatgcattcagagtctatcccacaggggttctcatcagtagctttacagttgcaacggggtatttcagataagtctgcagtgaagatctgtaccctgccaataggacggtttacctttatatgtttataaggtggtggcttcttgtcattctttcggtcttcctgcagctgtcttagctctttttgggcctttaattcctcaaaccttgctgcagcttcctgaagagcttttttatatgtcccatccactcctttgcccatcttatccttgctgctcacgtcaccctccatgtaagggaagactcgggcctggtgagtccacaaatagtcattagatccaaaaaagaggactgggaactctcccacatcatgtctcatcttatcaatgttggaaggaacagctcgaggatggcagatctcagctggccaccacctgtatcgtccaacttttacccagacaatctccctgtagtgtggctttttgcctgctttacagtcattgcaataccagtttccttcagggatatcaatgttcaggcattcacgatgaaaagcagcagggcaagaatcacagcacagaaggctgcctccttctgagcacacaaagcaccagctaacattaacatgctcatgatttcggcagccccgcctaggggtaaagtgattagggcagatgatactattagatgcaaggatctttgacccagcagccaggcaaaagtcattggcgtggtatgccacaggacagcggacacagcgcatcaaccgacctttagatgcagaaacattggctggattagcagcatgacaggttatacagatgtggagggagcaccggaagcccttgttctgcataacagtgggtgggtacttctggacacactcttcatggtaaaactttccacacaagggtagaaggcaccttttaacatcttccccactctgcttacatacaaaacaggtatggattcctgtgcgacattcattgcagataaattttcctcttggcatctcagtcaatccaaggcactccaggtggaaagccccacagcactgagcctcacataacagcagctcacccaatttttcacaattctgacagacattctccttgagtgcagctcctccaccgcgttcaccctgcatttttttagaggcaggcatcccgggatcgtgttctacaccttcctcaacagtctccttggggcttgtggccgtcctgtgaggcattagttctccctctgagcctggaatctcttttgacgagtcatcatttttcacttttttacactgcatcttggctgcagcatgcctctgtcgttttcgcttccttggcttgtcaaatatcttggtagtgcctccaccaaaatcttttgaataagatgtggcacaagattcagttatgccattctccaggtgaccagcttcatagcactttttagaaaggccaaggtcccccttcttgggcataaatccagggtctaaatcattggattcaagaagtttcttagttggttttctttgacgtttactttcataatttcctggcgttttaactagcaattcctcagactcaagggcaggccgtggagagacttccggagccacaggcacagacaaggtcagctgcggcaactcagcatgtccacctccaagttctgactgagccaaggggccctccaaaaacggagcctccctttcaagaactggaggctcttctttggttgaaatcaaagaattctcgtccacctgcttgttctgagcactagatcgacctcgggctagaaggctttcctcttcacagcgggaacttaccttgtgcacctgctcctgtaccttcttttgttttttcttaggagcaaatatctgatcatattcttctgtatattccaaaagccacttgcttggcttcctaaggcgtttcttctctgaccgcacagctggttcagggagctcagcctgtggtgtcaaactgggaattcctggctccttttccatgtcaccaatgctggcactggatttatcacaaacatttaaccgtggcccagctgaatctaagcagtcagcatgattttgctctgtcagtggttcctcaagtatgcttgctgaaggagttctatgctctggaaactcatcccgcccctcctgcacagggtcactaggaagtaagaccctaaaggcacactcagagttttctttctctttaaatctgttcatgcgcttacgaggtttagtgcgcctttggtttaaacgctgccaccgctttttaggcaccacttgatttacaccattgagttcatcattctcactgttcattacagagtccagctctgggccttttccgttttcaaaagagagtcctttttcagaaattttaccaggatcagattgcttaaccttgctatcgaaatgcacatcagaaaaatggtcaccatcttcacttgttaagtggcccattatctgaaggggatcctctttactaggatcttctgccccacctctcaatgaacctccacgttctcggtctccctgcagtacagcatcaagagtcacacttggaagctgattcagttttcttttgcgctcggtctttaaggctttacggttcactgtgttctttaccatttgggctgaaaaagcatctcgcaatttggatgaaggctttgatcgtccacagttgcgcctagtaacacagtctgaacgacttttaccagaagcagggaggtctctcttgtcggacagtaagccaggtagggaagcagacaactcgccagataatgcagagtcacccccactagggctaggattggcggagttctgagtgccatctccctttttctctgaattgtgtgtggagcctcctgaaaccaaaaccttagagactcctacaggactattagtagaacagtccccacgaccaggactccggtaagagaccaggttttgagcagtcatcaaccgctgctccttcgtcttactatcatgcatatctttcaacatcattagcaatgtactgaatttgtagtctggttcaataggtatgtgattctgactagaagcagaagagaaaagtaatggttttgatggctttgatgttccagagtcactgacatcctcacctaaggatctgtaagagagttccttcaactcggataaaacatgtttcaccactgctgtttctatgtcacttgaatccctggttttctcatgcatattgttcagtagttttagaccatccactttcccacttttagaaatgctggccaaaggagagcctttggtatcagaagagcagcatttcaaactgcactcctcatttataactgggggttctgccataactggattttctttgtgtttgcactttatacttcggaacttgggctgtttgcttttcgaatgtaatagagcttgatttgctgccccaccctttattaacgagttctcactggatatgcttgatgacaggttgaattttggagagagagcatcatttgtaaaatctgactggggtttgtgaacaagagtagatgccttcagatcagagagattaacctgagacgtctcggttccaggctctgcactcttagtacaacccattaagtggtctgtatgtgagttactaatgagaggcttctgttttgcttttaccctagtgtttgtggcagcaaacctagaatactttatcttttcatttttctgcatagataacatgttctctgttctatcgaaagcatctggaatttcaaggacactgttatcagactctgagctgtgttctatgggatccaggtcactgcttccatcatcagaagtggtacagatactaatggaatcacttcgcttttcctcatcacctgctccaatatagcagagcttcacttttgaaccacacaccaggcttcgttggggtttattcttctctcgagaacactttgagatcaaagcaccctcaggcaagcccaataaagagtcaccatttgaagtctcaaattctttctttgcagtgttttttccacaggaagaaaacagaaaacttcctggggcagtgttggaccctgtgaggctatttgctatcctggaaagttcattagaggcctgcgtatcagatatatccccagagataaagtttaggccaaggttctctggaatctttcccctccgttcatctttatgtgcttcaaattgtatgtggccctttttcacactagtcctttttggattatcagagctctttctggctcgagatttagcgcaaggcttttccttctcatctgcagaatgttcagaatcaaaagccagtgatttcaaacagccattaagcaacaggtcatgttctgactcaggatcatttgtgcagtcttcaaatggcatatcttcttcactgtccaacttgattgaaccaggaatacattttcggttctttgaccccttgggaacatcatactgttctgcaagtccaacactggcttcccatttactcaaaattttctgaggaaccttatgcctatatcctttttctttctgtttccctcttctcctaaggacaggtagctcttcgaattgatgtctgccttcaaacatgacgattgcttttccagccacccaggctctctcagaaggatctccaaaagcctccacgtagtactgccgatagggcctccggttggaaactttcatttttgaatgtgtgttaatcaacggatcagaacaaatcctgcagggccaccatgggcgtctcttgaattttgcccagatgagatctccaacttcatacttcagtggcgtagactttttcttaggttgacaaaatggcaattcctgtgaagtagatgatgatgaagttccaggtaattctagcatgtttcctaatgtactggtactggaatctggatcatccgaaagggctgtccttgtcttcaggggcatctaaattcactggattggaaaagggcagcagacaatttcttctgggtagttcacaggtctgatccatcctgggccggcatcaacctgaggggaggcggagg

SEQ ID NO: 19166 - RNA, 11340 nt, Homo sapiens
  source 1..11340: mol_type = other RNA
tgtcttctctcctcccaaacaggaacccgggtttcttgagctgccagtccctcaacccttggcagtgcttatttataccgtgaaattagcaccatcattacattttattgtgtgtgtgtacaaaacaatgatctattcttatttcaatttacactatagcagcctctggccctgttgcactggccctaggaagctcagctgagaactaactggccatagccaatgacaggctcccacagcaactaccaagcagtgacttggaatgtctacacatggaactgctcaaatgaaactcagcaagaaaggggctggaggcagctccttctctgccatgatctgagagaggttaggacactgggctcctctaacctggctgataaaccccaagaggatgacagtatcatttaaaaaaccttagtaaaatccaccttatagggactaagggtaaaacctatccaagtttcatgctgtcctcattactccctatgggggaatctgtcaggactaaactttctgccattctgttctcatgaggcaacattagaattacaacctgggagtccggctccagtgagcagacagtgccgagcctgggaagggatcaacagggtgtttcatgccctgaccatagtgtggggtgaaggatgtaaagaataaaataactattttcatcaatgctaaagatttggttcagaagagggtcaacacagtgatttaagtcatctcaaactcagtaacagggtaaagcagacatttaaaaatgaggatgtttctgtatcaatgacagctattttgctattagactgggttggctccagcaagataagcaaatgaggctttgaatgtaaatttcaacatttttcataatctttttctgacttagcagggctagatgtattggctttctagctacccatggagaatttcaacttttgccttgtccctggaaaaggcctcctggggagctggctccaaggcaaacactcttgagatctcaatttccaagcacatacccaaataccaccctgcgttaaggaccagaagttttctaagatgaaagatttccttttcactccaattcacatccctttggaaaaggggtcttattacaaacttcaggggacgtcccacagggctggcaaggccactccctccccaccttcctccaagagtcacatttcccaacagttgttgtgactctgcttctaattggatagtgactgctttcatgattttaaccatctagtatcacatgctgctactggtgggcccaatagctcaaatttctagtttccagtggttttctagttcccattcaatggcccttgaaggaagcccagatgtccatccattcagatgaagaactgctccccaaaatggctcagaagctgttttcccaggcaggtctggaacgaagcctccaatgaatggcggagaatggaaagaaccaaaataaaaccacaaagcagccaatcatggcccctttccctcactccctcctgtcctgtgagacatctagactgctgtcaagttgattacctaccaaagcctactttagagaagctactttagaatcaaacttctccacggaaaatttttacatggcctgcacgccctccccccgccccccccaaattcacagtttatttcatgaaacaaagagctacggtaatttaacacacaacatagtgaaaggagactctgacagtgcagtgcagatacctttttctgatcacaactacagatgactggagagaaaagggcacaggactggcaccaagcaaaccctactcatatgacctaaaagattagggaaagggacctactagctgcagttatatatttattattctcacacatgataaatacttaatataatgaactttaatgttctcggtgaatttctttaaaaatatctttttcatggtttaaaattcttttaaaagaaaataagatgctttacgttttctcttccttttgaacaaagagcttttcctctttgatgatgtgggaagagagagaggatgaaaggggagaactaggcaggtggaattcacagaggagattccgaggtctcagtgaaatgcagggataggcccctaaactcaggacagccctgcccagcctcgtccctctgcctgagttcaagtgtctcaacctcagagacagactttgggaaataaaagcagattctatttttaatctttagataaagcgcaaatgcttctataataactactgttccctccgtggaattgatgggagtaacctcaataagaacttgaggaaattgggaccaaatacagaatcctattgagagcgtgaaagccataactaagagataatggccaggagacgttagggccggggatggcctgctggctaagttggcaaagcagagaggtaaacatgttggtctaaggacaaaggaggggtagacaagtgggaggaaactagccaaacagcacttcctgttggcagtctgtgagctgggtgaatggtagggcagggtagcaccaacagatttcccagcccttgggccccagctcagggcagcagtaacagataatcagcagttaataggagtcatctcttagcctggacgttgctctaaacaccacctcttgccagtcttcagggaagggttctggcttgcctttgagctaagtcagcaggcaggtgctctcaatacagagcacagcaattctcagggaggcgaagaagaggactccctccactcaggagggaaaaggaatggggaaaagaaatttcccatcaggatctggtactcttcctgaagctggtgtgtctagctcagagcttgccagagattccctatgtccactgcccgaggctctgaaatctgaaagcacctgagtgttttagggaaatagggatggggtggattcatgtacaaagagaaaaataggtagaaacaaaagcaaagaaagagaagcttgccaaatgccttcttccactgctggaaatctacattcgcacagagcccgactgcccctgaccacctgctcctccaaggactgatcttgagactctgcacagcccagacaaaagcagcagcggcgaccccacagccaacagccttgctggcctcaatgcagcacccttgcatctatagaggagacctctgtgagtgtgcgcgcatgcacacgcacccatgcacaccgcagccaagagacacttcctcaacacaaccacttctggtgccacaaaggacatttcaaaatgagtctaaagccccagggcccctcagaacttcctgttacttcctggtcaaaggttcctgaaagccttggaatccaggctcacagggatgaggcctgtatctctcatcagtgactagcacccggcctagaacacgtgaatgctcaggaaatcgccactgatttgaaagaacaccatttcctcccaagggttcctaggtgccctcaatggggctctgtctggttggggaaatcgctttgagagcccctataccttccaacctgaccagcggaattgaattccatacttgactccagagtggactttttatttcacgatgaccatgtggaaaagttgggggaaagagacccaagtctgtctgtctccttggttggggcccactggattttcatacatggttcacacaaccataagcccccactggctaatgtcacaagagttctgagtgttgggatatgaggaaagaataacagtgggaaagtgttcggggcagatgtgtttttttttaagggggaaagaaagaaaagatttcccctccccaaatggtaccctgggggcagcttgtttgttcatgtgacattgattggtactacttctgttctgattctgcacacttgtgactggaaggagcctggttaagagctggaagtgtattttgctctggtttggggtcttgccctcttccaagagaccagcaagtctgtgccaatgtctgtgtgctcccagcagaccagcaagactgtgccagtgtctgtccagccactatgggccagagccctgcccgtgatgaggcttttcccagggcccagggactttgctctgtggttaccaacttcttttcttcagtggggagggaggctggggccttcccgagagacctaaaagattgcccactcttggcggcaagtgcaggtagttgctggcctccgaccatctgcttcgcctgcttcaccaggcccggggattggctaagaggccctggggtctgctcagcccctgcagaagctcttcctgaggcctgagttgttggctcatataaaaaggccttggcaggaggctgagaaagaagtctggcctgggtgagtgatttaacagcttgccaggggtcctctgaaggggctgctgctttcccagatgtctgaagaggatctgacacacagcctttctcaacagctctcggcatatgccccagacctttgctggcaggccatgaacttgactccaacactggcatcttctcatcagcctgtggtgtgacctgatgaggtgaagctgcccgctccttctggcgaggagttaggtctatgagatccatcaccaaagcagctctattttttgactgagtattctggtccacaggcctcagtgctttttctttagctacaagggtctggaccacagctgatagtactttctcaggaggtgggagtctctgggacaaagaggcatggggtttgtcagtaggcctgtctgaagtctggggtttgggactgctagtaatgagcagtctgtctggcggcggaagtctcaggccagtgggaactgaggttttctccagtgactggggccttgggctggcagcacctatggatttatccagccttgggtcagccgtccccagaggtctttccagtggttgggacctgactgagggtgaggagcttgggctggtcactggagagggtttgtcgcttagctggggtcttggtcctgccactgctggtggcctgtccagtggcctctggctggaaaccaaggattgggatttggtccctgacccagcgaggtctctgaccttatctaaaggctggggcctggagtcagttctctcaagaggtctttcaggtagcaatggcctctgacaagtccctgccagagcttttttggagagcgacagcatctggttggtgtcagcaggaggtttatctgacattttgggtgcctgagcagccattcctgttgattgctctgccaggtgagtgcttggccctggaggcagcggtactgggggaggcacatactcacggatctccccaggttccagaggattgggcccacaggggtcatgctcagtacaagacagacgcccatccagtttggaaatgaaaagcatcccttctcgatgctgcttacaaaaggagctggggcacatctcacagaaggaggctgcttccttcccgcagatgtcacactgatgccacggacattcccatttccctgctggtcgcttggtcagattgagacagtctgcgtggtaaacttttgggcagcctggtttcttgcaggagacgagctggccagcatccccacaactaaaacactcatcttctcgctcctttgtgatttcaccctgggtcctgcgctttccctgttgcttcttcttgaatttctttgacttttcttccgtggcaatgggttgattctttggccttacacccaagaagccactgcagttcggggctccacatttgcaaacagtctttccattcccaagacattctaggttgtagttgaaggtaagttcagtgcctgctttaatgtcacttagtgcaaaaaggcctacacgggtatctccattcacagaccacttctgtgtttcacagttgggctggcagcaatgattcatgaaccgagcatagtttcctttgggaccagcatcaatgattcggtctttgtctagggtgagcatatagaaattagtgatatcatgttcttgagcatagcgaattcgagctctgcattcttcttcatctataagctcacccacatactcattcacaaattcaccctttttaatatctgtttttgtccgtagaccccaaccccgctgtaatgtgcggaaaatttcaacctctggatattggcgcttggaaaagcactggttttgacagcgccctccggcaggacacactgtggggtggcactcatagagcagcatgcggttgatgcattcagagtctatcccacaggggttctcatcagtagctttacagttgcaacggggtatttcagataagtctgcagtgaagatctgtaccctgccaataggacggtttacctttatatgtttataaggtggtggcttcttgtcattctttcggtcttcctgcagctgtcttagctctttttgggcctttaattcctcaaaccttgctgcagcttcctgaagagcttttttatatgtcccatccactcctttgcccatcttatccttgctgctcacgtcaccctccatgtaagggaagactcgggcctggtgagtccacaaatagtcattagatccaaaaaagaggactgggaactctcccacatcatgtctcatcttatcaatgttggaaggaacagctcgaggatggcagatctcagctggccaccacctgtatcgtccaacttttacccagacaatctccctgtagtgtggctttttgcctgctttacagtcattgcaataccagtttccttcagggatatcaatgttcaggcattcacgatgaaaagcagcagggcaagaatcacagcacagaaggctgcctccttctgagcacacaaagcaccagctaacattaacatgctcatgatttcggcagccccgcctaggggtaaagtgattagggcagatgatactattagatgcaaggatctttgacccagcagccaggcaaaagtcattggcgtggtatgccacaggacagcggacacagcgcatcaaccgacctttagatgcagaaacattggctggattagcagcatgacaggttatacagatgtggagggagcaccggaagcccttgttctgcataacagtgggtgggtacttctggacacactcttcatggtaaaactttccacacaagggtagaaggcaccttttaacatcttccccactctgcttacatacaaaacaggtatggattcctgtgcgacattcattgcagataaattttcctcttggcatctcagtcaatccaaggcactccaggtggaaagccccacagcactgagcctcacataacagcagctcacccaatttttcacaattctgacagacattctccttgagtgcagctcctccaccgcgttcaccctgcatttttttagaggcaggcatcccgggatcgtgttctacaccttcctcaacagtctccttggggcttgtggccgtcctgtgaggcattagttctccctctgagcctggaatctcttttgacgagtcatcatttttcacttttttacactgcatcttggctgcagcatgcctctgtcgttttcgcttccttggcttgtcaaatatcttggtagtgcctccaccaaaatcttttgaataagatgtggcacaagattcagttatgccattctccaggtgaccagcttcatagcactttttagaaaggccaaggtcccccttcttgggcataaatccagggtctaaatcattggattcaagaagtttcttagttggttttctttgacgtttactttcataatttcctggcgttttaactagcaattcctcagactcaagggcaggccgtggagagacttccggagccacaggcacagacaaggtcagctgcggcaactcagcatgtccacctccaagttctgactgagccaaggggccctccaaaaacggagcctccctttcaagaactggaggctcttctttggttgaaatcaaagaattctcgtccacctgcttgttctgagcactagatcgacctcgggctagaaggctttcctcttcacagcgggaacttaccttgtgcacctgctcctgtaccttcttttgttttttcttaggagcaaatatctgatcatattcttctgtatattccaaaagccacttgcttggcttcctaaggcgtttcttctctgaccgcacagctggttcagggagctcagcctgtggtgtcaaactgggaattcctggctccttttccatgtcaccaatgctggcactggatttatcacaaacatttaaccgtggcccagctgaatctaagcagtcagcatgattttgctctgtcagtggttcctcaagtatgcttgctgaaggagttctatgctctggaaactcatcccgcccctcctgcacagggtcactaggaagtaagaccctaaaggcacactcagagttttctttctctttaaatctgttcatgcgcttacgaggtttagtgcgcctttggtttaaacgctgccaccgctttttaggcaccacttgatttacaccattgagttcatcattctcactgttcattacagagtccagctctgggccttttccgttttcaaaagagagtcctttttcagaaattttaccaggatcagattgcttaaccttgctatcgaaatgcacatcagaaaaatggtcaccatcttcacttgttaagtggcccattatctgaaggggatcctctttactaggatcttctgccccacctctcaatgaacctccacgttctcggtctccctgcagtacagcatcaagagtcacacttggaagctgattcagttttcttttgcgctcggtctttaaggctttacggttcactgtgttctttaccatttgggctgaaaaagcatctcgcaatttggatgaaggctttgatcgtccacagttgcgcctagtaacacagtctgaacgacttttaccagaagcagggaggtctctcttgtcggacagtaagccaggtagggaagcagacaactcgccagataatgcagagtcacccccactagggctaggattggcggagttctgagtgccatctccctttttctctgaattgtgtgtggagcctcctgaaaccaaaaccttagagactcctacaggactattagtagaacagtccccacgaccaggactccggtaagagaccaggttttgagcagtcatcaaccgctgctccttcgtcttactatcatgcatatctttcaacatcattagcaatgtactgaatttgtagtctggttcaataggtatgtgattctgactagaagcagaagagaaaagtaatggttttgatggctttgatgttccagagtcactgacatcctcacctaaggatctgtaagagagttccttcaactcggataaaacatgtttcaccactgctgtttctatgtcacttgaatccctggttttctcatgcatattgttcagtagttttagaccatccactttcccacttttagaaatgctggccaaaggagagcctttggtatcagaagagcagcatttcaaactgcactcctcatttataactgggggttctgccataactggattttctttgtgtttgcactttatacttcggaacttgggctgtttgcttttcgaatgtaatagagcttgatttgctgccccaccctttattaacgagttctcactggatatgcttgatgacaggttgaattttggagagagagcatcatttgtaaaatctgactggggtttgtgaacaagagtagatgccttcagatcagagagattaacctgagacgtctcggttccaggctctgcactcttagtacaacccattaagtggtctgtatgtgagttactaatgagaggcttctgttttgcttttaccctagtgtttgtggcagcaaacctagaatactttatcttttcatttttctgcatagataacatgttctctgttctatcgaaagcatctggaatttcaaggacactgttatcagactctgagctgtgttctatgggatccaggtcactgcttccatcatcagaagtggtacagatactaatggaatcacttcgcttttcctcatcacctgctccaatatagcagagcttcacttttgaaccacacaccaggcttcgttggggtttattcttctctcgagaacactttgagatcaaagcaccctcaggcaagcccaataaagagtcaccatttgaagtctcaaattctttctttgcagtgttttttccacaggaagaaaacagaaaacttcctggggcagtgttggaccctgtgaggctatttgctatcctggaaagttcattagaggcctgcgtatcagatatatccccagagataaagtttaggccaaggttctctggaatctttcccctccgttcatctttatgtgcttcaaattgtatgtggccctttttcacactagtcctttttggattatcagagctctttctggctcgagatttagcgcaaggcttttccttctcatctgcagaatgttcagaatcaaaagccagtgatttcaaacagccattaagcaacaggtcatgttctgactcaggatcatttgtgcagtcttcaaatggcatatcttcttcactgtccaacttgattgaaccaggaatacattttcggttctttgaccccttgggaacatcatactgttctgcaagtccaacactggcttcccatttactcaaaattttctgaggaaccttatgcctatatcctttttctttctgtttccctcttctcctaaggacaggtagctcttcgaattgatgtctgccttcaaacatgacgattgcttttccagccacccaggctctctcagaaggatctccaaaagcctccacgtagtactgccgatagggcctccggttggaaactttcatttttgaatgtgtgttaatcaacggatcagaacaaatcctgcagggccaccatgggcgtctcttgaattttgcccagatgagatctccaacttcatacttcagtggcgtagactttttcttaggttgacaaaatggcaattcctgtgaagtagatgatgatgaagttccaggtaattctagcatgtttcctaatgtactggtactggaatctggatcatccgaaagggctgtccttgtcttcaggggcatctaaattcactggattggaaaagggcagcagacaatttcttctgggtagttcacaggtctgatccatcctgggccggcatcaacctgggggcttgggctggggtcttcgaggcctcaggccccgagcagacgcggccgcaggcgaaccccctacccggccgcaccccaaacccacaccaccaccaccaccaccaccacagaccaagctgagcaggaaacaaaat

SEQ ID NO: 19167 - RNA, 11256 nt, Homo sapiens
  source 1..11256: mol_type = other RNA
tgtcttctctcctcccaaacaggaacccgggtttcttgagctgccagtccctcaacccttggcagtgcttatttataccgtgaaattagcaccatcattacattttattgtgtgtgtgtacaaaacaatgatctattcttatttcaatttacactatagcagcctctggccctgttgcactggccctaggaagctcagctgagaactaactggccatagccaatgacaggctcccacagcaactaccaagcagtgacttggaatgtctacacatggaactgctcaaatgaaactcagcaagaaaggggctggaggcagctccttctctgccatgatctgagagaggttaggacactgggctcctctaacctggctgataaaccccaagaggatgacagtatcatttaaaaaaccttagtaaaatccaccttatagggactaagggtaaaacctatccaagtttcatgctgtcctcattactccctatgggggaatctgtcaggactaaactttctgccattctgttctcatgaggcaacattagaattacaacctgggagtccggctccagtgagcagacagtgccgagcctgggaagggatcaacagggtgtttcatgccctgaccatagtgtggggtgaaggatgtaaagaataaaataactattttcatcaatgctaaagatttggttcagaagagggtcaacacagtgatttaagtcatctcaaactcagtaacagggtaaagcagacatttaaaaatgaggatgtttctgtatcaatgacagctattttgctattagactgggttggctccagcaagataagcaaatgaggctttgaatgtaaatttcaacatttttcataatctttttctgacttagcagggctagatgtattggctttctagctacccatggagaatttcaacttttgccttgtccctggaaaaggcctcctggggagctggctccaaggcaaacactcttgagatctcaatttccaagcacatacccaaataccaccctgcgttaaggaccagaagttttctaagatgaaagatttccttttcactccaattcacatccctttggaaaaggggtcttattacaaacttcaggggacgtcccacagggctggcaaggccactccctccccaccttcctccaagagtcacatttcccaacagttgttgtgactctgcttctaattggatagtgactgctttcatgattttaaccatctagtatcacatgctgctactggtgggcccaatagctcaaatttctagtttccagtggttttctagttcccattcaatggcccttgaaggaagcccagatgtccatccattcagatgaagaactgctccccaaaatggctcagaagctgttttcccaggcaggtctggaacgaagcctccaatgaatggcggagaatggaaagaaccaaaataaaaccacaaagcagccaatcatggcccctttccctcactccctcctgtcctgtgagacatctagactgctgtcaagttgattacctaccaaagcctactttagagaagctactttagaatcaaacttctccacggaaaatttttacatggcctgcacgccctccccccgccccccccaaattcacagtttatttcatgaaacaaagagctacggtaatttaacacacaacatagtgaaaggagactctgacagtgcagtgcagatacctttttctgatcacaactacagatgactggagagaaaagggcacaggactggcaccaagcaaaccctactcatatgacctaaaagattagggaaagggacctactagctgcagttatatatttattattctcacacatgataaatacttaatataatgaactttaatgttctcggtgaatttctttaaaaatatctttttcatggtttaaaattcttttaaaagaaaataagatgctttacgttttctcttccttttgaacaaagagcttttcctctttgatgatgtgggaagagagagaggatgaaaggggagaactaggcaggtggaattcacagaggagattccgaggtctcagtgaaatgcagggataggcccctaaactcaggacagccctgcccagcctcgtccctctgcctgagttcaagtgtctcaacctcagagacagactttgggaaataaaagcagattctatttttaatctttagataaagcgcaaatgcttctataataactactgttccctccgtggaattgatgggagtaacctcaataagaacttgaggaaattgggaccaaatacagaatcctattgagagcgtgaaagccataactaagagataatggccaggagacgttagggccggggatggcctgctggctaagttggcaaagcagagaggtaaacatgttggtctaaggacaaaggaggggtagacaagtgggaggaaactagccaaacagcacttcctgttggcagtctgtgagctgggtgaatggtagggcagggtagcaccaacagatttcccagcccttgggccccagctcagggcagcagtaacagataatcagcagttaataggagtcatctcttagcctggacgttgctctaaacaccacctcttgccagtcttcagggaagggttctggcttgcctttgagctaagtcagcaggcaggtgctctcaatacagagcacagcaattctcagggaggcgaagaagaggactccctccactcaggagggaaaaggaatggggaaaagaaatttcccatcaggatctggtactcttcctgaagctggtgtgtctagctcagagcttgccagagattccctatgtccactgcccgaggctctgaaatctgaaagcacctgagtgttttagggaaatagggatggggtggattcatgtacaaagagaaaaataggtagaaacaaaagcaaagaaagagaagcttgccaaatgccttcttccactgctggaaatctacattcgcacagagcccgactgcccctgaccacctgctcctccaaggactgatcttgagactctgcacagcccagacaaaagcagcagcggcgaccccacagccaacagccttgctggcctcaatgcagcacccttgcatctatagaggagacctctgtgagtgtgcgcgcatgcacacgcacccatgcacaccgcagccaagagacacttcctcaacacaaccacttctggtgccacaaaggacatttcaaaatgagtctaaagccccagggcccctcagaacttcctgttacttcctggtcaaaggttcctgaaagccttggaatccaggctcacagggatgaggcctgtatctctcatcagtgactagcacccggcctagaacacgtgaatgctcaggaaatcgccactgatttgaaagaacaccatttcctcccaagggttcctaggtgccctcaatggggctctgtctggttggggaaatcgctttgagagcccctataccttccaacctgaccagcggaattgaattccatacttgactccagagtggactttttatttcacgatgaccatgtggaaaagttgggggaaagagacccaagtctgtctgtctccttggttggggcccactggattttcatacatggttcacacaaccataagcccccactggctaatgtcacaagagttctgagtgttgggatatgaggaaagaataacagtgggaaagtgttcggggcagatgtgtttttttttaagggggaaagaaagaaaagatttcccctccccaaatggtaccctgggggcagcttgtttgttcatgtgacattgattggtactacttctgttctgattctgcacacttgtgactggaaggagcctggttaagagctggaagtgtattttgctctggtttggggtcttgccctcttccaagagaccagcaagtctgtgccaatgtctgtgtgctcccagcagaccagcaagactgtgccagtgtctgtccagccactatgggccagagccctgcccgtgatgaggcttttcccagggcccagggactttgctctgtggttaccaacttcttttcttcagtggggagggaggctggggccttcccgagagacctaaaagattgcccactcttggcggcaagtgcaggtagttgctggcctccgaccatctgcttcgcctgcttcaccaggcccggggattggctaagaggccctggggtctgctcagcccctgcagaagctcttcctgaggcctgagttgttggctcatataaaaaggccttggcaggaggctgagaaagaagtctggcctgggtgagtgatttaacagcttgccaggggtcctctgaaggggctgctgctttcccagatgtctgaagaggatctgacacacagcctttctcaacagctctcggcatatgccccagacctttgctggcaggccatgaacttgactccaacactggcatcttctcatcagcctgtggtgtgacctgatgaggtgaagctgcccgctccttctggcgaggagttaggtctatgagatccatcaccaaagcagctctattttttgactgagtattctggtccacaggcctcagtgctttttctttagctacaagggtctggaccacagctgatagtactttctcaggaggtgggagtctctgggacaaagaggcatggggtttgtcagtaggcctgtctgaagtctggggtttgggactgctagtaatgagcagtctgtctggcggcggaagtctcaggccagtgggaactgaggttttctccagtgactggggccttgggctggcagcacctatggatttatccagccttgggtcagccgtccccagaggtctttccagtggttgggacctgactgagggtgaggagcttgggctggtcactggagagggtttgtcgcttagctggggtcttggtcctgccactgctggtggcctgtccagtggcctctggctggaaaccaaggattgggatttggtccctgacccagcgaggtctctgaccttatctaaaggctggggcctggagtcagttctctcaagaggtctttcaggtagcaatggcctctgacaagtccctgccagagcttttttggagagcgacagcatctggttggtgtcagcaggaggtttatctgacattttgggtgcctgagcagccattcctgttgattgctctgccaggtgagtgcttggccctggaggcagcggtactgggggaggcacatactcacggatctccccaggttccagaggattgggcccacaggggtcatgctcagtacaagacagacgcccatccagtttggaaatgaaaagcatcccttctcgatgctgcttacaaaaggagctggggcacatctcacagaaggaggctgcttccttcccgcagatgtcacactgatgccacggacattcccatttccctgctggtcgcttggtcagattgagacagtctgcgtggtaaacttttgggcagcctggtttcttgcaggagacgagctggccagcatccccacaactaaaacactcatcttctcgctcctttgtgatttcaccctgggtcctgcgctttccctgttgcttcttcttgaatttctttgacttttcttccgtggcaatgggttgattctttggccttacacccaagaagccactgcagttcggggctccacatttgcaaacagtctttccattcccaagacattctaggttgtagttgaaggtaagttcagtgcctgctttaatgtcacttagtgcaaaaaggcctacacgggtatctccattcacagaccacttctgtgtttcacagttgggctggcagcaatgattcatgaaccgagcatagtttcctttgggaccagcatcaatgattcggtctttgtctagggtgagcatatagaaattagtgatatcatgttcttgagcatagcgaattcgagctctgcattcttcttcatctataagctcacccacatactcattcacaaattcaccctttttaatatctgtttttgtccgtagaccccaaccccgctgtaatgtgcggaaaatttcaacctctggatattggcgcttggaaaagcactggttttgacagcgccctccggcaggacacactgtggggtggcactcatagagcagcatgcggttgatgcattcagagtctatcccacaggggttctcatcagtagctttacagttgcaacggggtatttcagataagtctgcagtgaagatctgtaccctgccaataggacggtttacctttatatgtttataaggtggtggcttcttgtcattctttcggtcttcctgcagctgtcttagctctttttgggcctttaattcctcaaaccttgctgcagcttcctgaagagcttttttatatgtcccatccactcctttgcccatcttatccttgctgctcacgtcaccctccatgtaagggaagactcgggcctggtgagtccacaaatagtcattagatccaaaaaagaggactgggaactctcccacatcatgtctcatcttatcaatgttggaaggaacagctcgaggatggcagatctcagctggccaccacctgtatcgtccaacttttacccagacaatctccctgtagtgtggctttttgcctgctttacagtcattgcaataccagtttccttcagggatatcaatgttcaggcattcacgatgaaaagcagcagggcaagaatcacagcacagaaggctgcctccttctgagcacacaaagcaccagctaacattaacatgctcatgatttcggcagccccgcctaggggtaaagtgattagggcagatgatactattagatgcaaggatctttgacccagcagccaggcaaaagtcattggcgtggtatgccacaggacagcggacacagcgcatcaaccgacctttagatgcagaaacattggctggattagcagcatgacaggttatacagatgtggagggagcaccggaagcccttgttctgcataacagtgggtgggtacttctggacacactcttcatggtaaaactttccacacaagggtagaaggcaccttttaacatcttccccactctgcttacatacaaaacaggtatggattcctgtgcgacattcattgcagataaattttcctcttggcatctcagtcaatccaaggcactccaggtggaaagccccacagcactgagcctcacataacagcagctcacccaatttttcacaattctgacagacattctccttgagtgcagctcctccaccgcgttcaccctgcatttttttagaggcaggcatcccgggatcgtgttctacaccttcctcaacagtctccttggggcttgtggccgtcctgtgaggcattagttctccctctgagcctggaatctcttttgacgagtcatcatttttcacttttttacactgcatcttggctgcagcatgcctctgtcgttttcgcttccttggcttgtcaaatatcttggtagtgcctccaccaaaatcttttgaataagatgtggcacaagattcagttatgccattctccaggtgaccagcttcatagcactttttagaaaggccaaggtcccccttcttgggcataaatccagggtctaaatcattggattcaagaagtttcttagttggttttctttgacgtttactttcataatttcctggcgttttaactagcaattcctcagactcaagggcaggccgtggagagacttccggagccacaggcacagacaaggtcagctgcggcaactcagcatgtccacctccaagttctgactgagccaaggggccctccaaaaacggagcctccctttcaagaactggaggctcttctttggttgaaatcaaagaattctcgtccacctgcttgttctgagcactagatcgacctcgggctagaaggctttcctcttcacagcgggaacttaccttgtgcacctgctcctgtaccttcttttgttttttcttaggagcaaatatctgatcatattcttctgtatattccaaaagccacttgcttggcttcctaaggcgtttcttctctgaccgcacagctggttcagggagctcagcctgtggtgtcaaactgggaattcctggctccttttccatgtcaccaatgctggcactggatttatcacaaacatttaaccgtggcccagctgaatctaagcagtcagcatgattttgctctgtcagtggttcctcaagtatgcttgctgaaggagttctatgctctggaaactcatcccgcccctcctgcacagggtcactaggaagtaagaccctaaaggcacactcagagttttctttctctttaaatctgttcatgcgcttacgaggtttagtgcgcctttggtttaaacgctgccaccgctttttaggcaccacttgatttacaccattgagttcatcattctcactgttcattacagagtccagctctgggccttttccgttttcaaaagagagtcctttttcagaaattttaccaggatcagattgcttaaccttgctatcgaaatgcacatcagaaaaatggtcaccatcttcacttgttaagtggcccattatctgaaggggatcctctttactaggatcttctgccccacctctcaatgaacctccacgttctcggtctccctgcagtacagcatcaagagtcacacttggaagctgattcagttttcttttgcgctcggtctttaaggctttacggttcactgtgttctttaccatttgggctgaaaaagcatctcgcaatttggatgaaggctttgatcgtccacagttgcgcctagtaacacagtctgaacgacttttaccagaagcagggaggtctctcttgtcggacagtaagccaggtagggaagcagacaactcgccagataatgcagagtcacccccactagggctaggattggcggagttctgagtgccatctccctttttctctgaattgtgtgtggagcctcctgaaaccaaaaccttagagactcctacaggactattagtagaacagtccccacgaccaggactccggtaagagaccaggttttgagcagtcatcaaccgctgctccttcgtcttactatcatgcatatctttcaacatcattagcaatgtactgaatttgtagtctggttcaataggtatgtgattctgactagaagcagaagagaaaagtaatggttttgatggctttgatgttccagagtcactgacatcctcacctaaggatctgtaagagagttccttcaactcggataaaacatgtttcaccactgctgtttctatgtcacttgaatccctggttttctcatgcatattgttcagtagttttagaccatccactttcccacttttagaaatgctggccaaaggagagcctttggtatcagaagagcagcatttcaaactgcactcctcatttataactgggggttctgccataactggattttctttgtgtttgcactttatacttcggaacttgggctgtttgcttttcgaatgtaatagagcttgatttgctgccccaccctttattaacgagttctcactggatatgcttgatgacaggttgaattttggagagagagcatcatttgtaaaatctgactggggtttgtgaacaagagtagatgccttcagatcagagagattaacctgagacgtctcggttccaggctctgcactcttagtacaacccattaagtggtctgtatgtgagttactaatgagaggcttctgttttgcttttaccctagtgtttgtggcagcaaacctagaatactttatcttttcatttttctgcatagataacatgttctctgttctatcgaaagcatctggaatttcaaggacactgttatcagactctgagctgtgttctatgggatccaggtcactgcttccatcatcagaagtggtacagatactaatggaatcacttcgcttttcctcatcacctgctccaatatagcagagcttcacttttgaaccacacaccaggcttcgttggggtttattcttctctcgagaacactttgagatcaaagcaccctcaggcaagcccaataaagagtcaccatttgaagtctcaaattctttctttgcagtgttttttccacaggaagaaaacagaaaacttcctggggcagtgttggaccctgtgaggctatttgctatcctggaaagttcattagaggcctgcgtatcagatatatccccagagataaagtttaggccaaggttctctggaatctttcccctccgttcatctttatgtgcttcaaattgtatgtggccctttttcacactagtcctttttggattatcagagctctttctggctcgagatttagcgcaaggcttttccttctcatctgcagaatgttcagaatcaaaagccagtgatttcaaacagccattaagcaacaggtcatgttctgactcaggatcatttgtgcagtcttcaaatggcatatcttcttcactgtccaacttgattgaaccaggaatacattttcggttctttgaccccttgggaacatcatactgttctgcaagtccaacactggcttcccatttactcaaaattttctgaggaaccttatgcctatatcctttttctttctgtttccctcttctcctaaggacaggtagctcttcgaattgatgtctgccttcaaacatgacgattgcttttccagccacccaggctctctcagaaggatctccaaaagcctccacgtagtactgccgatagggcctccggttggaaactttcatttttgaatgtgtgttaatcaacggatcagaacaaatcctgcagggccaccatgggcgtctcttgaattttgcccagatgagatctccaacttcatacttcagtggcgtagactttttcttaggttgacaaaatggcaattcctgtgaagtagatgatgatgaagttccaggtaattctagcatgtttcctaatgtactggtactggaatctggatcatccgaaagggctgtccttgtcttcaggggcatctaaattcactggattggaaaagggcagcagacaatttcttctgggtagttcacaggtctgatccatcctgggccggcatcaactcttcggggttcagggcgggtgaagtcgggcttgtgagagcgccgcccaatcagcg

SEQ ID NO: 19168 - RNA, 12120 nt, Homo sapiens
  source 1..12120: mol_type = other RNA
tgtcttctctcctcccaaacaggaacccgggtttcttgagctgccagtccctcaacccttggcagtgcttatttataccgtgaaattagcaccatcattacattttattgtgtgtgtgtacaaaacaatgatctattcttatttcaatttacactatagcagcctctggccctgttgcactggccctaggaagctcagctgagaactaactggccatagccaatgacaggctcccacagcaactaccaagcagtgacttggaatgtctacacatggaactgctcaaatgaaactcagcaagaaaggggctggaggcagctccttctctgccatgatctgagagaggttaggacactgggctcctctaacctggctgataaaccccaagaggatgacagtatcatttaaaaaaccttagtaaaatccaccttatagggactaagggtaaaacctatccaagtttcatgctgtcctcattactccctatgggggaatctgtcaggactaaactttctgccattctgttctcatgaggcaacattagaattacaacctgggagtccggctccagtgagcagacagtgccgagcctgggaagggatcaacagggtgtttcatgccctgaccatagtgtggggtgaaggatgtaaagaataaaataactattttcatcaatgctaaagatttggttcagaagagggtcaacacagtgatttaagtcatctcaaactcagtaacagggtaaagcagacatttaaaaatgaggatgtttctgtatcaatgacagctattttgctattagactgggttggctccagcaagataagcaaatgaggctttgaatgtaaatttcaacatttttcataatctttttctgacttagcagggctagatgtattggctttctagctacccatggagaatttcaacttttgccttgtccctggaaaaggcctcctggggagctggctccaaggcaaacactcttgagatctcaatttccaagcacatacccaaataccaccctgcgttaaggaccagaagttttctaagatgaaagatttccttttcactccaattcacatccctttggaaaaggggtcttattacaaacttcaggggacgtcccacagggctggcaaggccactccctccccaccttcctccaagagtcacatttcccaacagttgttgtgactctgcttctaattggatagtgactgctttcatgattttaaccatctagtatcacatgctgctactggtgggcccaatagctcaaatttctagtttccagtggttttctagttcccattcaatggcccttgaaggaagcccagatgtccatccattcagatgaagaactgctccccaaaatggctcagaagctgttttcccaggcaggtctggaacgaagcctccaatgaatggcggagaatggaaagaaccaaaataaaaccacaaagcagccaatcatggcccctttccctcactccctcctgtcctgtgagacatctagactgctgtcaagttgattacctaccaaagcctactttagagaagctactttagaatcaaacttctccacggaaaatttttacatggcctgcacgccctccccccgccccccccaaattcacagtttatttcatgaaacaaagagctacggtaatttaacacacaacatagtgaaaggagactctgacagtgcagtgcagatacctttttctgatcacaactacagatgactggagagaaaagggcacaggactggcaccaagcaaaccctactcatatgacctaaaagattagggaaagggacctactagctgcagttatatatttattattctcacacatgataaatacttaatataatgaactttaatgttctcggtgaatttctttaaaaatatctttttcatggtttaaaattcttttaaaagaaaataagatgctttacgttttctcttccttttgaacaaagagcttttcctctttgatgatgtgggaagagagagaggatgaaaggggagaactaggcaggtggaattcacagaggagattccgaggtctcagtgaaatgcagggataggcccctaaactcaggacagccctgcccagcctcgtccctctgcctgagttcaagtgtctcaacctcagagacagactttgggaaataaaagcagattctatttttaatctttagataaagcgcaaatgcttctataataactactgttccctccgtggaattgatgggagtaacctcaataagaacttgaggaaattgggaccaaatacagaatcctattgagagcgtgaaagccataactaagagataatggccaggagacgttagggccggggatggcctgctggctaagttggcaaagcagagaggtaaacatgttggtctaaggacaaaggaggggtagacaagtgggaggaaactagccaaacagcacttcctgttggcagtctgtgagctgggtgaatggtagggcagggtagcaccaacagatttcccagcccttgggccccagctcagggcagcagtaacagataatcagcagttaataggagtcatctcttagcctggacgttgctctaaacaccacctcttgccagtcttcagggaagggttctggcttgcctttgagctaagtcagcaggcaggtgctctcaatacagagcacagcaattctcagggaggcgaagaagaggactccctccactcaggagggaaaaggaatggggaaaagaaatttcccatcaggatctggtactcttcctgaagctggtgtgtctagctcagagcttgccagagattccctatgtccactgcccgaggctctgaaatctgaaagcacctgagtgttttagggaaatagggatggggtggattcatgtacaaagagaaaaataggtagaaacaaaagcaaagaaagagaagcttgccaaatgccttcttccactgctggaaatctacattcgcacagagcccgactgcccctgaccacctgctcctccaaggactgatcttgagactctgcacagcccagacaaaagcagcagcggcgaccccacagccaacagccttgctggcctcaatgcagcacccttgcatctatagaggagacctctgtgagtgtgcgcgcatgcacacgcacccatgcacaccgcagccaagagacacttcctcaacacaaccacttctggtgccacaaaggacatttcaaaatgagtctaaagccccagggcccctcagaacttcctgttacttcctggtcaaaggttcctgaaagccttggaatccaggctcacagggatgaggcctgtatctctcatcagtgactagcacccggcctagaacacgtgaatgctcaggaaatcgccactgatttgaaagaacaccatttcctcccaagggttcctaggtgccctcaatggggctctgtctggttggggaaatcgctttgagagcccctataccttccaacctgaccagcggaattgaattccatacttgactccagagtggactttttatttcacgatgaccatgtggaaaagttgggggaaagagacccaagtctgtctgtctccttggttggggcccactggattttcatacatggttcacacaaccataagcccccactggctaatgtcacaagagttctgagtgttgggatatgaggaaagaataacagtgggaaagtgttcggggcagatgtgtttttttttaagggggaaagaaagaaaagatttcccctccccaaatggtaccctgggggcagcttgtttgttcatgtgacattgattggtactacttctgttctgattctgcacacttgtgactggaaggagcctggttaagagctggaagtgtattttgctctggtttggggtcttgccctcttccaagagaccagcaagtctgtgccaatgtctgtgtgctcccagcagaccagcaagactgtgccagtgtctgtccagccactatgggccagagccctgcccgtgatgaggcttttcccagggcccagggactttgctctgtggttaccaacttcttttcttcagtggggagggaggctggggccttcccgagagacctaaaagattgcccactcttggcggcaagtgcaggtagttgctggcctccgaccatctgcttcgcctgcttcaccaggcccggggattggctaagaggccctggggtctgctcagcccctgcagaagctcttcctgaggcctgagttgttggctcatataaaaaggccttggcaggaggctgagaaagaagtctggcctgggtgagtgatttaacagcttgccaggggtcctctgaaggggctgctgctttcccagatgtctgaagaggatctgacacacagcctttctcaacagctctcggcatatgccccagacctttgctggcaggccatgaacttgactccaacactggcatcttctcatcagcctgtggtgtgacctgatgaggtgaagctgcccgctccttctggcgaggagttaggtctatgagatccatcaccaaagcagctctattttttgactgagtattctggtccacaggcctcagtgctttttctttagctacaagggtctggaccacagctgatagtactttctcaggaggtgggagtctctgggacaaagaggcatggggtttgtcagtaggcctgtctgaagtctggggtttgggactgctagtaatgagcagtctgtctggcggcggaagtctcaggccagtgggaactgaggttttctccagtgactggggccttgggctggcagcacctatggatttatccagccttgggtcagccgtccccagaggtctttccagtggttgggacctgactgagggtgaggagcttgggctggtcactggagagggtttgtcgcttagctggggtcttggtcctgccactgctggtggcctgtccagtggcctctggctggaaaccaaggattgggatttggtccctgacccagcgaggtctctgaccttatctaaaggctggggcctggagtcagttctctcaagaggtctttcaggtagcaatggcctctgacaagtccctgccagagcttttttggagagcgacagcatctggttggtgtcagcaggaggtttatctgacattttgggtgcctgagcagccattcctgttgattgctctgccaggtgagtgcttggccctggaggcagcggtactgggggaggcacatactcacggatctccccaggttccagaggattgggcccacaggggtcatgctcagtacaagacagacgcccatccagtttggaaatgaaaagcatcccttctcgatgctgcttacaaaaggagctggggcacatctcacagaaggaggctgcttccttcccgcagatgtcacactgatgccacggacattcccatttccctgctggtcgcttggtcagattgagacagtctgcgtggtaaacttttgggcagcctggtttcttgcaggagacgagctggccagcatccccacaactaaaacactcatcttctcgctcctttgtgatttcaccctgggtcctgcgctttccctgttgcttcttcttgaatttctttgacttttcttccgtggcaatgggttgattctttggccttacacccaagaagccactgcagttcggggctccacatttgcaaacagtctttccattcccaagacattctaggttgtagttgaaggtaagttcagtgcctgctttaatgtcacttagtgcaaaaaggcctacacgggtatctccattcacagaccacttctgtgtttcacagttgggctggcagcaatgattcatgaaccgagcatagtttcctttgggaccagcatcaatgattcggtctttgtctagggtgagcatatagaaattagtgatatcatgttcttgagcatagcgaattcgagctctgcattcttcttcatctataagctcacccacatactcattcacaaattcaccctttttaatatctgtttttgtccgtagaccccaaccccgctgtaatgtgcggaaaatttcaacctctggatattggcgcttggaaaagcactggttttgacagcgccctccggcaggacacactgtggggtggcactcatagagcagcatgcggttgatgcattcagagtctatcccacaggggttctcatcagtagctttacagttgcaacggggtatttcagataagtctgcagtgaagatctgtaccctgccaataggacggtttacctttatatgtttataaggtggtggcttcttgtcattctttcggtcttcctgcagctgtcttagctctttttgggcctttaattcctcaaaccttgctgcagcttcctgaagagcttttttatatgtcccatccactcctttgcccatcttatccttgctgctcacgtcaccctccatgtaagggaagactcgggcctggtgagtccacaaatagtcattagatccaaaaaagaggactgggaactctcccacatcatgtctcatcttatcaatgttggaaggaacagctcgaggatggcagatctcagctggccaccacctgtatcgtccaacttttacccagacaatctccctgtagtgtggctttttgcctgctttacagtcattgcaataccagtttccttcagggatatcaatgttcaggcattcacgatgaaaagcagcagggcaagaatcacagcacagaaggctgcctccttctgagcacacaaagcaccagctaacattaacatgctcatgatttcggcagccccgcctaggggtaaagtgattagggcagatgatactattagatgcaaggatctttgacccagcagccaggcaaaagtcattggcgtggtatgccacaggacagcggacacagcgcatcaaccgacctttagatgcagaaacattggctggattagcagcatgacaggttatacagatgtggagggagcaccggaagcccttgttctgcataacagtgggtgggtacttctggacacactcttcatggtaaaactttccacacaagggtagaaggcaccttttaacatcttccccactctgcttacatacaaaacaggtatggattcctgtgcgacattcattgcagataaattttcctcttggcatctcagtcaatccaaggcactccaggtggaaagccccacagcactgagcctcacataacagcagctcacccaatttttcacaattctgacagacattctccttgagtgcagctcctccaccgcgttcaccctgcatttttttagaggcaggcatcccgggatcgtgttctacaccttcctcaacagtctccttggggcttgtggccgtcctgtgaggcattagttctccctctgagcctggaatctcttttgacgagtcatcatttttcacttttttacactgcatcttggctgcagcatgcctctgtcgttttcgcttccttggcttgtcaaatatcttggtagtgcctccaccaaaatcttttgaataagatgtggcacaagattcagttatgccattctccaggtgaccagcttcatagcactttttagaaaggccaaggtcccccttcttgggcataaatccagggtctaaatcattggattcaagaagtttcttagttggttttctttgacgtttactttcataatttcctggcgttttaactagcaattcctcagactcaagggcaggccgtggagagacttccggagccacaggcacagacaaggtcagctgcggcaactcagcatgtccacctccaagttctgactgagccaaggggccctccaaaaacggagcctccctttcaagaactggaggctcttctttggttgaaatcaaagaattctcgtccacctgcttgttctgagcactagatcgacctcgggctagaaggctttcctcttcacagcgggaacttaccttgtgcacctgctcctgtaccttcttttgttttttcttaggagcaaatatctgatcatattcttctgtatattccaaaagccacttgcttggcttcctaaggcgtttcttctctgaccgcacagctggttcagggagctcagcctgtggtgtcaaactgggaattcctggctccttttccatgtcaccaatgctggcactggatttatcacaaacatttaaccgtggcccagctgaatctaagcagtcagcatgattttgctctgtcagtggttcctcaagtatgcttgctgaaggagttctatgctctggaaactcatcccgcccctcctgcacagggtcactaggaagtaagaccctaaaggcacactcagagttttctttctctttaaatctgttcatgcgcttacgaggtttagtgcgcctttggtttaaacgctgccaccgctttttaggcaccacttgatttacaccattgagttcatcattctcactgttcattacagagtccagctctgggccttttccgttttcaaaagagagtcctttttcagaaattttaccaggatcagattgcttaaccttgctatcgaaatgcacatcagaaaaatggtcaccatcttcacttgttaagtggcccattatctgaaggggatcctctttactaggatcttctgccccacctctcaatgaacctccacgttctcggtctccctgcagtacagcatcaagagtcacacttggaagctgattcagttttcttttgcgctcggtctttaaggctttacggttcactgtgttctttaccatttgggctgaaaaagcatctcgcaatttggatgaaggctttgatcgtccacagttgcgcctagtaacacagtctgaacgacttttaccagaagcagggaggtctctcttgtcggacagtaagccaggtagggaagcagacaactcgccagataatgcagagtcacccccactagggctaggattggcggagttctgagtgccatctccctttttctctgaattgtgtgtggagcctcctgaaaccaaaaccttagagactcctacaggactattagtagaacagtccccacgaccaggactccggtaagagaccaggttttgagcagtcatcaaccgctgctccttcgtcttactatcatgcatatctttcaacatcattagcaatgtactgaatttgtagtctggttcaataggtatgtgattctgactagaagcagaagagaaaagtaatggttttgatggctttgatgttccagagtcactgacatcctcacctaaggatctgtaagagagttccttcaactcggataaaacatgtttcaccactgctgtttctatgtcacttgaatccctggttttctcatgcatattgttcagtagttttagaccatccactttcccacttttagaaatgctggccaaaggagagcctttggtatcagaagagcagcatttcaaactgcactcctcatttataactgggggttctgccataactggattttctttgtgtttgcactttatacttcggaacttgggctgtttgcttttcgaatgtaatagagcttgatttgctgccccaccctttattaacgagttctcactggatatgcttgatgacaggttgaattttggagagagagcatcatttgtaaaatctgactggggtttgtgaacaagagtagatgccttcagatcagagagattaacctgagacgtctcggttccaggctctgcactcttagtacaacccattaagtggtctgtatgtgagttactaatgagaggcttctgttttgcttttaccctagtgtttgtggcagcaaacctagaatactttatcttttcatttttctgcatagataacatgttctctgttctatcgaaagcatctggaatttcaaggacactgttatcagactctgagctgtgttctatgggatccaggtcactgcttccatcatcagaagtggtacagatactaatggaatcacttcgcttttcctcatcacctgctccaatatagcagagcttcacttttgaaccacacaccaggcttcgttggggtttattcttctctcgagaacactttgagatcaaagcaccctcaggcaagcccaataaagagtcaccatttgaagtctcaaattctttctttgcagtgttttttccacaggaagaaaacagaaaacttcctggggcagtgttggaccctgtgaggctatttgctatcctggaaagttcattagaggcctgcgtatcagatatatccccagagataaagtttaggccaaggttctctggaatctttcccctccgttcatctttatgtgcttcaaattgtatgtggccctttttcacactagtcctttttggattatcagagctctttctggctcgagatttagcgcaaggcttttccttctcatctgcagaatgttcagaatcaaaagccagtgatttcaaacagccattaagcaacaggtcatgttctgactcaggatcatttgtgcagtcttcaaatggcatatcttcttcactgtccaacttgattgaaccaggaatacattttcggttctttgaccccttgggaacatcatactgttctgcaagtccaacactggcttcccatttactcaaaattttctgaggaaccttatgcctatatcctttttctttctgtttccctcttctcctaaggacaggtagctcttcgaattgatgtctgccttcaaacatgacgattgcttttccagccacccaggctctctcagaaggatctccaaaagcctccacgtagtactgccgatagggcctccggttggaaactttcatttttgaatgtgtgttaatcaacggatcagaacaaatcctgcagggccaccatgggcgtctcttgaattttgcccagatgagatctccaacttcatacttcagtggcgtagactttttcttaggttgacaaaatggcaattcctgtgaagtagatgatgatgaagttccaggtaattctagcatgtttcctaatgtactggtactggaatctggatcatcctgaaaagataaatttattgagtttaattgctcttctattgtaatgtttgtgtctcctagtgaaaagggggctgggagaagggctgctttttcattgctgccgtccacttcatttctttgcttatttttctgtgtttcagtctgaggagctaatggcaagaatggcgatttgactgcaccgtgtctactctctggtgtgctgtcttgttcacttcccatggccacttttacaccattctctgatttagtctcataattgcaggtggcattggtctgagtttcctcaaagatctcctctatactctcatcctctgtgactggctgttctgggtccatttcagaatctacatctgcatcgtccacacaagtaaaattctcaaagtgcagaaagccattcttgatagtctttgttacttttacctggagttcaggggagttattacaagagggttcctgtttcatagcaagtgctgtaggaccaccaggactcaaggaagtgcaaacaattggcgtctgagctcttgaatcacttttttcagggtcttgaaaggattctgatccatcagcagacccatttaaatactctacattgatcatggaggccaaatcctgtagtctccgcagtggaatgtaacaagatggagaatcttgtccataagcattttgggatgttccactgacagtcgataactgcatagtacacccattaagtggctcagaaaaattggattgaccattaccgaaagggctgtccttgtcttcaggggcatctaaattcactggattggaaaagggcagcagacaatttcttctgggtagttcacaggtctgatccatcctgggccggcatcaaccgtgccccgcgccccctcccgggccagctggggggagggggtgaccctcattacactggggtgcgagcggagcggtggggagagagcggggccgctcgccgcacccccctccccccgcgtctctcttcaggggagaaggcagcgagcgcgacctgccccggcctattccgccgccgcctc

SEQ ID NO: 19169 - RNA, 12694 nt, Homo sapiens
  source 1..12694: mol_type = other RNA
tgtcttctctcctcccaaacaggaacccgggtttcttgagctgccagtccctcaacccttggcagtgcttatttataccgtgaaattagcaccatcattacattttattgtgtgtgtgtacaaaacaatgatctattcttatttcaatttacactatagcagcctctggccctgttgcactggccctaggaagctcagctgagaactaactggccatagccaatgacaggctcccacagcaactaccaagcagtgacttggaatgtctacacatggaactgctcaaatgaaactcagcaagaaaggggctggaggcagctccttctctgccatgatctgagagaggttaggacactgggctcctctaacctggctgataaaccccaagaggatgacagtatcatttaaaaaaccttagtaaaatccaccttatagggactaagggtaaaacctatccaagtttcatgctgtcctcattactccctatgggggaatctgtcaggactaaactttctgccattctgttctcatgaggcaacattagaattacaacctgggagtccggctccagtgagcagacagtgccgagcctgggaagggatcaacagggtgtttcatgccctgaccatagtgtggggtgaaggatgtaaagaataaaataactattttcatcaatgctaaagatttggttcagaagagggtcaacacagtgatttaagtcatctcaaactcagtaacagggtaaagcagacatttaaaaatgaggatgtttctgtatcaatgacagctattttgctattagactgggttggctccagcaagataagcaaatgaggctttgaatgtaaatttcaacatttttcataatctttttctgacttagcagggctagatgtattggctttctagctacccatggagaatttcaacttttgccttgtccctggaaaaggcctcctggggagctggctccaaggcaaacactcttgagatctcaatttccaagcacatacccaaataccaccctgcgttaaggaccagaagttttctaagatgaaagatttccttttcactccaattcacatccctttggaaaaggggtcttattacaaacttcaggggacgtcccacagggctggcaaggccactccctccccaccttcctccaagagtcacatttcccaacagttgttgtgactctgcttctaattggatagtgactgctttcatgattttaaccatctagtatcacatgctgctactggtgggcccaatagctcaaatttctagtttccagtggttttctagttcccattcaatggcccttgaaggaagcccagatgtccatccattcagatgaagaactgctccccaaaatggctcagaagctgttttcccaggcaggtctggaacgaagcctccaatgaatggcggagaatggaaagaaccaaaataaaaccacaaagcagccaatcatggcccctttccctcactccctcctgtcctgtgagacatctagactgctgtcaagttgattacctaccaaagcctactttagagaagctactttagaatcaaacttctccacggaaaatttttacatggcctgcacgccctccccccgccccccccaaattcacagtttatttcatgaaacaaagagctacggtaatttaacacacaacatagtgaaaggagactctgacagtgcagtgcagatacctttttctgatcacaactacagatgactggagagaaaagggcacaggactggcaccaagcaaaccctactcatatgacctaaaagattagggaaagggacctactagctgcagttatatatttattattctcacacatgataaatacttaatataatgaactttaatgttctcggtgaatttctttaaaaatatctttttcatggtttaaaattcttttaaaagaaaataagatgctttacgttttctcttccttttgaacaaagagcttttcctctttgatgatgtgggaagagagagaggatgaaaggggagaactaggcaggtggaattcacagaggagattccgaggtctcagtgaaatgcagggataggcccctaaactcaggacagccctgcccagcctcgtccctctgcctgagttcaagtgtctcaacctcagagacagactttgggaaataaaagcagattctatttttaatctttagataaagcgcaaatgcttctataataactactgttccctccgtggaattgatgggagtaacctcaataagaacttgaggaaattgggaccaaatacagaatcctattgagagcgtgaaagccataactaagagataatggccaggagacgttagggccggggatggcctgctggctaagttggcaaagcagagaggtaaacatgttggtctaaggacaaaggaggggtagacaagtgggaggaaactagccaaacagcacttcctgttggcagtctgtgagctgggtgaatggtagggcagggtagcaccaacagatttcccagcccttgggccccagctcagggcagcagtaacagataatcagcagttaataggagtcatctcttagcctggacgttgctctaaacaccacctcttgccagtcttcagggaagggttctggcttgcctttgagctaagtcagcaggcaggtgctctcaatacagagcacagcaattctcagggaggcgaagaagaggactccctccactcaggagggaaaaggaatggggaaaagaaatttcccatcaggatctggtactcttcctgaagctggtgtgtctagctcagagcttgccagagattccctatgtccactgcccgaggctctgaaatctgaaagcacctgagtgttttagggaaatagggatggggtggattcatgtacaaagagaaaaataggtagaaacaaaagcaaagaaagagaagcttgccaaatgccttcttccactgctggaaatctacattcgcacagagcccgactgcccctgaccacctgctcctccaaggactgatcttgagactctgcacagcccagacaaaagcagcagcggcgaccccacagccaacagccttgctggcctcaatgcagcacccttgcatctatagaggagacctctgtgagtgtgcgcgcatgcacacgcacccatgcacaccgcagccaagagacacttcctcaacacaaccacttctggtgccacaaaggacatttcaaaatgagtctaaagccccagggcccctcagaacttcctgttacttcctggtcaaaggttcctgaaagccttggaatccaggctcacagggatgaggcctgtatctctcatcagtgactagcacccggcctagaacacgtgaatgctcaggaaatcgccactgatttgaaagaacaccatttcctcccaagggttcctaggtgccctcaatggggctctgtctggttggggaaatcgctttgagagcccctataccttccaacctgaccagcggaattgaattccatacttgactccagagtggactttttatttcacgatgaccatgtggaaaagttgggggaaagagacccaagtctgtctgtctccttggttggggcccactggattttcatacatggttcacacaaccataagcccccactggctaatgtcacaagagttctgagtgttgggatatgaggaaagaataacagtgggaaagtgttcggggcagatgtgtttttttttaagggggaaagaaagaaaagatttcccctccccaaatggtaccctgggggcagcttgtttgttcatgtgacattgattggtactacttctgttctgattctgcacacttgtgactggaaggagcctggttaagagctggaagtgtattttgctctggtttggggtcttgccctcttccaagagaccagcaagtctgtgccaatgtctgtgtgctcccagcagaccagcaagactgtgccagtgtctgtccagccactatgggccagagccctgcccgtgatgaggcttttcccagggcccagggactttgctctgtggttaccaacttcttttcttcagtggggagggaggctggggccttcccgagagacctaaaagattgcccactcttggcggcaagtgcaggtagttgctggcctccgaccatctgcttcgcctgcttcaccaggcccggggattggctaagaggccctggggtctgctcagcccctgcagaagctcttcctgaggcctgagttgttggctcatataaaaaggccttggcaggaggctgagaaagaagtctggcctgggtgagtgatttaacagcttgccaggggtcctctgaaggggctgctgctttcccagatgtctgaagaggatctgacacacagcctttctcaacagctctcggcatatgccccagacctttgctggcaggccatgaacttgactccaacactggcatcttctcatcagcctgtggtgtgacctgatgaggtgaagctgcccgctccttctggcgaggagttaggtctatgagatccatcaccaaagcagctctattttttgactgagtattctggtccacaggcctcagtgctttttctttagctacaagggtctggaccacagctgatagtactttctcaggaggtgggagtctctgggacaaagaggcatggggtttgtcagtaggcctgtctgaagtctggggtttgggactgctagtaatgagcagtctgtctggcggcggaagtctcaggccagtgggaactgaggttttctccagtgactggggccttgggctggcagcacctatggatttatccagccttgggtcagccgtccccagaggtctttccagtggttgggacctgactgagggtgaggagcttgggctggtcactggagagggtttgtcgcttagctggggtcttggtcctgccactgctggtggcctgtccagtggcctctggctggaaaccaaggattgggatttggtccctgacccagcgaggtctctgaccttatctaaaggctggggcctggagtcagttctctcaagaggtctttcaggtagcaatggcctctgacaagtccctgccagagcttttttggagagcgacagcatctggttggtgtcagcaggaggtttatctgacattttgggtgcctgagcagccattcctgttgattgctctgccaggtgagtgcttggccctggaggcagcggtactgggggaggcacatactcacggatctccccaggttccagaggattgggcccacaggggtcatgctcagtacaagacagacgcccatccagtttggaaatgaaaagcatcccttctcgatgctgcttacaaaaggagctggggcacatctcacagaaggaggctgcttccttcccgcagatgtcacactgatgccacggacattcccatttccctgctggtcgcttggtcagattgagacagtctgcgtggtaaacttttgggcagcctggtttcttgcaggagacgagctggccagcatccccacaactaaaacactcatcttctcgctcctttgtgatttcaccctgggtcctgcgctttccctgttgcttcttcttgaatttctttgacttttcttccgtggcaatgggttgattctttggccttacacccaagaagccactgcagttcggggctccacatttgcaaacagtctttccattcccaagacattctaggttgtagttgaaggtaagttcagtgcctgctttaatgtcacttagtgcaaaaaggcctacacgggtatctccattcacagaccacttctgtgtttcacagttgggctggcagcaatgattcatgaaccgagcatagtttcctttgggaccagcatcaatgattcggtctttgtctagggtgagcatatagaaattagtgatatcatgttcttgagcatagcgaattcgagctctgcattcttcttcatctataagctcacccacatactcattcacaaattcaccctttttaatatctgtttttgtccgtagaccccaaccccgctgtaatgtgcggaaaatttcaacctctggatattggcgcttggaaaagcactggttttgacagcgccctccggcaggacacactgtggggtggcactcatagagcagcatgcggttgatgcattcagagtctatcccacaggggttctcatcagtagctttacagttgcaacggggtatttcagataagtctgcagtgaagatctgtaccctgccaataggacggtttacctttatatgtttataaggtggtggcttcttgtcattctttcggtcttcctgcagctgtcttagctctttttgggcctttaattcctcaaaccttgctgcagcttcctgaagagcttttttatatgtcccatccactcctttgcccatcttatccttgctgctcacgtcaccctccatgtaagggaagactcgggcctggtgagtccacaaatagtcattagatccaaaaaagaggactgggaactctcccacatcatgtctcatcttatcaatgttggaaggaacagctcgaggatggcagatctcagctggccaccacctgtatcgtccaacttttacccagacaatctccctgtagtgtggctttttgcctgctttacagtcattgcaataccagtttccttcagggatatcaatgttcaggcattcacgatgaaaagcagcagggcaagaatcacagcacagaaggctgcctccttctgagcacacaaagcaccagctaacattaacatgctcatgatttcggcagccccgcctaggggtaaagtgattagggcagatgatactattagatgcaaggatctttgacccagcagccaggcaaaagtcattggcgtggtatgccacaggacagcggacacagcgcatcaaccgacctttagatgcagaaacattggctggattagcagcatgacaggttatacagatgtggagggagcaccggaagcccttgttctgcataacagtgggtgggtacttctggacacactcttcatggtaaaactttccacacaagggtagaaggcaccttttaacatcttccccactctgcttacatacaaaacaggtatggattcctgtgcgacattcattgcagataaattttcctcttggcatctcagtcaatccaaggcactccaggtggaaagccccacagcactgagcctcacataacagcagctcacccaatttttcacaattctgacagacattctccttgagtgcagctcctccaccgcgttcaccctgcatttttttagaggcaggcatcccgggatcgtgttctacaccttcctcaacagtctccttggggcttgtggccgtcctgtgaggcattagttctccctctgagcctggaatctcttttgacgagtcatcatttttcacttttttacactgcatcttggctgcagcatgcctctgtcgttttcgcttccttggcttgtcaaatatcttggtagtgcctccaccaaaatcttttgaataagatgtggcacaagattcagttatgccattctccaggtgaccagcttcatagcactttttagaaaggccaaggtcccccttcttgggcataaatccagggtctaaatcattggattcaagaagtttcttagttggttttctttgacgtttactttcataatttcctggcgttttaactagcaattcctcagactcaagggcaggccgtggagagacttccggagccacaggcacagacaaggtcagctgcggcaactcagcatgtccacctccaagttctgactgagccaaggggccctccaaaaacggagcctccctttcaagaactggaggctcttctttggttgaaatcaaagaattctcgtccacctgcttgttctgagcactagatcgacctcgggctagaaggctttcctcttcacagcgggaacttaccttgtgcacctgctcctgtaccttcttttgttttttcttaggagcaaatatctgatcatattcttctgtatattccaaaagccacttgcttggcttcctaaggcgtttcttctctgaccgcacagctggttcagggagctcagcctgtggtgtcaaactgggaattcctggctccttttccatgtcaccaatgctggcactggatttatcacaaacatttaaccgtggcccagctgaatctaagcagtcagcatgattttgctctgtcagtggttcctcaagtatgcttgctgaaggagttctatgctctggaaactcatcccgcccctcctgcacagggtcactaggaagtaagaccctaaaggcacactcagagttttctttctctttaaatctgttcatgcgcttacgaggtttagtgcgcctttggtttaaacgctgccaccgctttttaggcaccacttgatttacaccattgagttcatcattctcactgttcattacagagtccagctctgggccttttccgttttcaaaagagagtcctttttcagaaattttaccaggatcagattgcttaaccttgctatcgaaatgcacatcagaaaaatggtcaccatcttcacttgttaagtggcccattatctgaaggggatcctctttactaggatcttctgccccacctctcaatgaacctccacgttctcggtctccctgcagtacagcatcaagagtcacacttggaagctgattcagttttcttttgcgctcggtctttaaggctttacggttcactgtgttctttaccatttgggctgaaaaagcatctcgcaatttggatgaaggctttgatcgtccacagttgcgcctagtaacacagtctgaacgacttttaccagaagcagggaggtctctcttgtcggacagtaagccaggtagggaagcagacaactcgccagataatgcagagtcacccccactagggctaggattggcggagttctgagtgccatctccctttttctctgaattgtgtgtggagcctcctgaaaccaaaaccttagagactcctacaggactattagtagaacagtccccacgaccaggactccggtaagagaccaggttttgagcagtcatcaaccgctgctccttcgtcttactatcatgcatatctttcaacatcattagcaatgtactgaatttgtagtctggttcaataggtatgtgattctgactagaagcagaagagaaaagtaatggttttgatggctttgatgttccagagtcactgacatcctcacctaaggatctgtaagagagttccttcaactcggataaaacatgtttcaccactgctgtttctatgtcacttgaatccctggttttctcatgcatattgttcagtagttttagaccatccactttcccacttttagaaatgctggccaaaggagagcctttggtatcagaagagcagcatttcaaactgcactcctcatttataactgggggttctgccataactggattttctttgtgtttgcactttatacttcggaacttgggctgtttgcttttcgaatgtaatagagcttgatttgctgccccaccctttattaacgagttctcactggatatgcttgatgacaggttgaattttggagagagagcatcatttgtaaaatctgactggggtttgtgaacaagagtagatgccttcagatcagagagattaacctgagacgtctcggttccaggctctgcactcttagtacaacccattaagtggtctgtatgtgagttactaatgagaggcttctgttttgcttttaccctagtgtttgtggcagcaaacctagaatactttatcttttcatttttctgcatagataacatgttctctgttctatcgaaagcatctggaatttcaaggacactgttatcagactctgagctgtgttctatgggatccaggtcactgcttccatcatcagaagtggtacagatactaatggaatcacttcgcttttcctcatcacctgctccaatatagcagagcttcacttttgaaccacacaccaggcttcgttggggtttattcttctctcgagaacactttgagatcaaagcaccctcaggcaagcccaataaagagtcaccatttgaagtctcaaattctttctttgcagtgttttttccacaggaagaaaacagaaaacttcctggggcagtgttggaccctgtgaggctatttgctatcctggaaagttcattagaggcctgcgtatcagatatatccccagagataaagtttaggccaaggttctctggaatctttcccctccgttcatctttatgtgcttcaaattgtatgtggccctttttcacactagtcctttttggattatcagagctctttctggctcgagatttagcgcaaggcttttccttctcatctgcagaatgttcagaatcaaaagccagtgatttcaaacagccattaagcaacaggtcatgttctgactcaggatcatttgtgcagtcttcaaatggcatatcttcttcactgtccaacttgattgaaccaggaatacattttcggttctttgaccccttgggaacatcatactgttctgcaagtccaacactggcttcccatttactcaaaattttctgaggaaccttatgcctatatcctttttctttctgtttccctcttctcctaaggacaggtagctcttcgaattgatgtctgccttcaaacatgacgattgcttttccagccacccaggctctctcagaaggatctccaaaagcctccacgtagtactgccgatagggcctccggttggaaactttcatttttgaatgtgtgttaatcaacggatcagaacaaatcctgcagggccaccatgggcgtctcttgaattttgcccagatgagatctccaacttcatacttcagtggcgtagactttttcttaggttgacaaaatggcaattcctgtgaagtagatgatgatgaagttccaggtaattctagcatgtttcctaatgtactggtactggaatctggatcatcctgaaaagataaatttattgagtttaattgctcttctattgtaatgtttgtgtctcctagtgaaaagggggctgggagaagggctgctttttcattgctgccgtccacttcatttctttgcttatttttctgtgtttcagtctgaggagctaatggcaagaatggcgatttgactgcaccgtgtctactctctggtgtgctgtcttgttcacttcccatggccacttttacaccattctctgatttagtctcataattgcaggtggcattggtctgagtttcctcaaagatctcctctatactctcatcctctgtgactggctgttctgggtccatttcagaatctacatctgcatcgtccacacaagtaaaattctcaaagtgcagaaagccattcttgatagtctttgttacttttacctggagttcaggggagttattacaagagggttcctgtttcatagcaagtgctgtaggaccaccaggactcaaggaagtgcaaacaattggcgtctgagctcttgaatcacttttttcagggtcttgaaaggattctgatccatcagcagacccatttaaatactctacattgatcatggaggccaaatcctgtagtctccgcagtggaatgtaacaagatggagaatcttgtccataagcattttgggatgttccactgacagtcgataactgcatagtacacccattaagtggctcagaaaaattggattgaccattaccgaaagggctgtccttgtcttcaggggcatctaaattcactggattggaaaagggcagcagacaatttcttctgggtagttcacaggtctgatccatcctgggccggcatcaacctcggggcacggcgctggcctcgggccgcacacggctcccgcaccctacgcgtctcgaaccccaacccaggcggcacctggcgcggctgaggcctgtccgatcgtcccgccagccctgctcgggcccgcgtcagtcccggcctccatcttaggttacagcccaggctccccatccactgggcacctgccctcagcccgctgggttcggcccgaggccaaggcaacccccctcctgccgcagggctcacctgggggcttgggctggggtcttcgaggcctcaggccccgagcagacgcggccgcaggcgaaccccctacccggccgcaccccaaacccacaccaccaccaccaccaccaccacagaccaagctgagcaggaaacaaaatggaggcagcagctcgggtctgcctccctgagccaagcctgtgcagccccagggctccctcctgtctcaggctcgacgcccgcgaggcagaggctggatcgtcccgggtgccgcgggcagccgccctacagcagcgcagacgggccggggactcggccctgcggtgcccacagcccctcacccaccaccccttcccttccccctccccccatccctctccctccccttgccgggccgtgcggggtgagcggctctggggagccgggtcgggttacccgccccggcactgctcgcccggccgtggcctccgcgggggaacgaagccaggcgaccccagcgctgagcccacccccggcaccgagccggg

SEQ ID NO: 19170 - RNA, 12045 nt, Homo sapiens
  source 1..12045: mol_type = other RNA
tgtcttctctcctcccaaacaggaacccgggtttcttgagctgccagtccctcaacccttggcagtgcttatttataccgtgaaattagcaccatcattacattttattgtgtgtgtgtacaaaacaatgatctattcttatttcaatttacactatagcagcctctggccctgttgcactggccctaggaagctcagctgagaactaactggccatagccaatgacaggctcccacagcaactaccaagcagtgacttggaatgtctacacatggaactgctcaaatgaaactcagcaagaaaggggctggaggcagctccttctctgccatgatctgagagaggttaggacactgggctcctctaacctggctgataaaccccaagaggatgacagtatcatttaaaaaaccttagtaaaatccaccttatagggactaagggtaaaacctatccaagtttcatgctgtcctcattactccctatgggggaatctgtcaggactaaactttctgccattctgttctcatgaggcaacattagaattacaacctgggagtccggctccagtgagcagacagtgccgagcctgggaagggatcaacagggtgtttcatgccctgaccatagtgtggggtgaaggatgtaaagaataaaataactattttcatcaatgctaaagatttggttcagaagagggtcaacacagtgatttaagtcatctcaaactcagtaacagggtaaagcagacatttaaaaatgaggatgtttctgtatcaatgacagctattttgctattagactgggttggctccagcaagataagcaaatgaggctttgaatgtaaatttcaacatttttcataatctttttctgacttagcagggctagatgtattggctttctagctacccatggagaatttcaacttttgccttgtccctggaaaaggcctcctggggagctggctccaaggcaaacactcttgagatctcaatttccaagcacatacccaaataccaccctgcgttaaggaccagaagttttctaagatgaaagatttccttttcactccaattcacatccctttggaaaaggggtcttattacaaacttcaggggacgtcccacagggctggcaaggccactccctccccaccttcctccaagagtcacatttcccaacagttgttgtgactctgcttctaattggatagtgactgctttcatgattttaaccatctagtatcacatgctgctactggtgggcccaatagctcaaatttctagtttccagtggttttctagttcccattcaatggcccttgaaggaagcccagatgtccatccattcagatgaagaactgctccccaaaatggctcagaagctgttttcccaggcaggtctggaacgaagcctccaatgaatggcggagaatggaaagaaccaaaataaaaccacaaagcagccaatcatggcccctttccctcactccctcctgtcctgtgagacatctagactgctgtcaagttgattacctaccaaagcctactttagagaagctactttagaatcaaacttctccacggaaaatttttacatggcctgcacgccctccccccgccccccccaaattcacagtttatttcatgaaacaaagagctacggtaatttaacacacaacatagtgaaaggagactctgacagtgcagtgcagatacctttttctgatcacaactacagatgactggagagaaaagggcacaggactggcaccaagcaaaccctactcatatgacctaaaagattagggaaagggacctactagctgcagttatatatttattattctcacacatgataaatacttaatataatgaactttaatgttctcggtgaatttctttaaaaatatctttttcatggtttaaaattcttttaaaagaaaataagatgctttacgttttctcttccttttgaacaaagagcttttcctctttgatgatgtgggaagagagagaggatgaaaggggagaactaggcaggtggaattcacagaggagattccgaggtctcagtgaaatgcagggataggcccctaaactcaggacagccctgcccagcctcgtccctctgcctgagttcaagtgtctcaacctcagagacagactttgggaaataaaagcagattctatttttaatctttagataaagcgcaaatgcttctataataactactgttccctccgtggaattgatgggagtaacctcaataagaacttgaggaaattgggaccaaatacagaatcctattgagagcgtgaaagccataactaagagataatggccaggagacgttagggccggggatggcctgctggctaagttggcaaagcagagaggtaaacatgttggtctaaggacaaaggaggggtagacaagtgggaggaaactagccaaacagcacttcctgttggcagtctgtgagctgggtgaatggtagggcagggtagcaccaacagatttcccagcccttgggccccagctcagggcagcagtaacagataatcagcagttaataggagtcatctcttagcctggacgttgctctaaacaccacctcttgccagtcttcagggaagggttctggcttgcctttgagctaagtcagcaggcaggtgctctcaatacagagcacagcaattctcagggaggcgaagaagaggactccctccactcaggagggaaaaggaatggggaaaagaaatttcccatcaggatctggtactcttcctgaagctggtgtgtctagctcagagcttgccagagattccctatgtccactgcccgaggctctgaaatctgaaagcacctgagtgttttagggaaatagggatggggtggattcatgtacaaagagaaaaataggtagaaacaaaagcaaagaaagagaagcttgccaaatgccttcttccactgctggaaatctacattcgcacagagcccgactgcccctgaccacctgctcctccaaggactgatcttgagactctgcacagcccagacaaaagcagcagcggcgaccccacagccaacagccttgctggcctcaatgcagcacccttgcatctatagaggagacctctgtgagtgtgcgcgcatgcacacgcacccatgcacaccgcagccaagagacacttcctcaacacaaccacttctggtgccacaaaggacatttcaaaatgagtctaaagccccagggcccctcagaacttcctgttacttcctggtcaaaggttcctgaaagccttggaatccaggctcacagggatgaggcctgtatctctcatcagtgactagcacccggcctagaacacgtgaatgctcaggaaatcgccactgatttgaaagaacaccatttcctcccaagggttcctaggtgccctcaatggggctctgtctggttggggaaatcgctttgagagcccctataccttccaacctgaccagcggaattgaattccatacttgactccagagtggactttttatttcacgatgaccatgtggaaaagttgggggaaagagacccaagtctgtctgtctccttggttggggcccactggattttcatacatggttcacacaaccataagcccccactggctaatgtcacaagagttctgagtgttgggatatgaggaaagaataacagtgggaaagtgttcggggcagatgtgtttttttttaagggggaaagaaagaaaagatttcccctccccaaatggtaccctgggggcagcttgtttgttcatgtgacattgattggtactacttctgttctgattctgcacacttgtgactggaaggagcctggttaagagctggaagtgtattttgctctggtttggggtcttgccctcttccaagagaccagcaagtctgtgccaatgtctgtgtgctcccagcagaccagcaagactgtgccagtgtctgtccagccactatgggccagagccctgcccgtgatgaggcttttcccagggcccagggactttgctctgtggttaccaacttcttttcttcagtggggagggaggctggggccttcccgagagacctaaaagattgcccactcttggcggcaagtgcaggtagttgctggcctccgaccatctgcttcgcctgcttcaccaggcccggggattggctaagaggccctggggtctgctcagcccctgcagaagctcttcctgaggcctgagttgttggctcatataaaaaggccttggcaggaggctgagaaagaagtctggcctgggtgagtgatttaacagcttgccaggggtcctctgaaggggctgctgctttcccagatgtctgaagaggatctgacacacagcctttctcaacagctctcggcatatgccccagacctttgctggcaggccatgaacttgactccaacactggcatcttctcatcagcctgtggtgtgacctgatgaggtgaagctgcccgctccttctggcgaggagttaggtctatgagatccatcaccaaagcagctctattttttgactgagtattctggtccacaggcctcagtgctttttctttagctacaagggtctggaccacagctgatagtactttctcaggaggtgggagtctctgggacaaagaggcatggggtttgtcagtaggcctgtctgaagtctggggtttgggactgctagtaatgagcagtctgtctggcggcggaagtctcaggccagtgggaactgaggttttctccagtgactggggccttgggctggcagcacctatggatttatccagccttgggtcagccgtccccagaggtctttccagtggttgggacctgactgagggtgaggagcttgggctggtcactggagagggtttgtcgcttagctggggtcttggtcctgccactgctggtggcctgtccagtggcctctggctggaaaccaaggattgggatttggtccctgacccagcgaggtctctgaccttatctaaaggctggggcctggagtcagttctctcaagaggtctttcaggtagcaatggcctctgacaagtccctgccagagcttttttggagagcgacagcatctggttggtgtcagcaggaggtttatctgacattttgggtgcctgagcagccattcctgttgattgctctgccaggtgagtgcttggccctggaggcagcggtactgggggaggcacatactcacggatctccccaggttccagaggattgggcccacaggggtcatgctcagtacaagacagacgcccatccagtttggaaatgaaaagcatcccttctcgatgctgcttacaaaaggagctggggcacatctcacagaaggaggctgcttccttcccgcagatgtcacactgatgccacggacattcccatttccctgctggtcgcttggtcagattgagacagtctgcgtggtaaacttttgggcagcctggtttcttgcaggagacgagctggccagcatccccacaactaaaacactcatcttctcgctcctttgtgatttcaccctgggtcctgcgctttccctgttgcttcttcttgaatttctttgacttttcttccgtggcaatgggttgattctttggccttacacccaagaagccactgcagttcggggctccacatttgcaaacagtctttccattcccaagacattctaggttgtagttgaaggtaagttcagtgcctgctttaatgtcacttagtgcaaaaaggcctacacgggtatctccattcacagaccacttctgtgtttcacagttgggctggcagcaatgattcatgaaccgagcatagtttcctttgggaccagcatcaatgattcggtctttgtctagggtgagcatatagaaattagtgatatcatgttcttgagcatagcgaattcgagctctgcattcttcttcatctataagctcacccacatactcattcacaaattcaccctttttaatatctgtttttgtccgtagaccccaaccccgctgtaatgtgcggaaaatttcaacctctggatattggcgcttggaaaagcactggttttgacagcgccctccggcaggacacactgtggggtggcactcatagagcagcatgcggttgatgcattcagagtctatcccacaggggttctcatcagtagctttacagttgcaacggggtatttcagataagtctgcagtgaagatctgtaccctgccaataggacggtttacctttatatgtttataaggtggtggcttcttgtcattctttcggtcttcctgcagctgtcttagctctttttgggcctttaattcctcaaaccttgctgcagcttcctgaagagcttttttatatgtcccatccactcctttgcccatcttatccttgctgctcacgtcaccctccatgtaagggaagactcgggcctggtgagtccacaaatagtcattagatccaaaaaagaggactgggaactctcccacatcatgtctcatcttatcaatgttggaaggaacagctcgaggatggcagatctcagctggccaccacctgtatcgtccaacttttacccagacaatctccctgtagtgtggctttttgcctgctttacagtcattgcaataccagtttccttcagggatatcaatgttcaggcattcacgatgaaaagcagcagggcaagaatcacagcacagaaggctgcctccttctgagcacacaaagcaccagctaacattaacatgctcatgatttcggcagccccgcctaggggtaaagtgattagggcagatgatactattagatgcaaggatctttgacccagcagccaggcaaaagtcattggcgtggtatgccacaggacagcggacacagcgcatcaaccgacctttagatgcagaaacattggctggattagcagcatgacaggttatacagatgtggagggagcaccggaagcccttgttctgcataacagtgggtgggtacttctggacacactcttcatggtaaaactttccacacaagggtagaaggcaccttttaacatcttccccactctgcttacatacaaaacaggtatggattcctgtgcgacattcattgcagataaattttcctcttggcatctcagtcaatccaaggcactccaggtggaaagccccacagcactgagcctcacataacagcagctcacccaatttttcacaattctgacagacattctccttgagtgcagctcctccaccgcgttcaccctgcatttttttagaggcaggcatcccgggatcgtgttctacaccttcctcaacagtctccttggggcttgtggccgtcctgtgaggcattagttctccctctgagcctggaatctcttttgacgagtcatcatttttcacttttttacactgcatcttggctgcagcatgcctctgtcgttttcgcttccttggcttgtcaaatatcttggtagtgcctccaccaaaatcttttgaataagatgtggcacaagattcagttatgccattctccaggtgaccagcttcatagcactttttagaaaggccaaggtcccccttcttgggcataaatccagggtctaaatcattggattcaagaagtttcttagttggttttctttgacgtttactttcataatttcctggcgttttaactagcaattcctcagactcaagggcaggccgtggagagacttccggagccacaggcacagacaaggtcagctgcggcaactcagcatgtccacctccaagttctgactgagccaaggggccctccaaaaacggagcctccctttcaagaactggaggctcttctttggttgaaatcaaagaattctcgtccacctgcttgttctgagcactagatcgacctcgggctagaaggctttcctcttcacagcgggaacttaccttgtgcacctgctcctgtaccttcttttgttttttcttaggagcaaatatctgatcatattcttctgtatattccaaaagccacttgcttggcttcctaaggcgtttcttctctgaccgcacagctggttcagggagctcagcctgtggtgtcaaactgggaattcctggctccttttccatgtcaccaatgctggcactggatttatcacaaacatttaaccgtggcccagctgaatctaagcagtcagcatgattttgctctgtcagtggttcctcaagtatgcttgctgaaggagttctatgctctggaaactcatcccgcccctcctgcacagggtcactaggaagtaagaccctaaaggcacactcagagttttctttctctttaaatctgttcatgcgcttacgaggtttagtgcgcctttggtttaaacgctgccaccgctttttaggcaccacttgatttacaccattgagttcatcattctcactgttcattacagagtccagctctgggccttttccgttttcaaaagagagtcctttttcagaaattttaccaggatcagattgcttaaccttgctatcgaaatgcacatcagaaaaatggtcaccatcttcacttgttaagtggcccattatctgaaggggatcctctttactaggatcttctgccccacctctcaatgaacctccacgttctcggtctccctgcagtacagcatcaagagtcacacttggaagctgattcagttttcttttgcgctcggtctttaaggctttacggttcactgtgttctttaccatttgggctgaaaaagcatctcgcaatttggatgaaggctttgatcgtccacagttgcgcctagtaacacagtctgaacgacttttaccagaagcagggaggtctctcttgtcggacagtaagccaggtagggaagcagacaactcgccagataatgcagagtcacccccactagggctaggattggcggagttctgagtgccatctccctttttctctgaattgtgtgtggagcctcctgaaaccaaaaccttagagactcctacaggactattagtagaacagtccccacgaccaggactccggtaagagaccaggttttgagcagtcatcaaccgctgctccttcgtcttactatcatgcatatctttcaacatcattagcaatgtactgaatttgtagtctggttcaataggtatgtgattctgactagaagcagaagagaaaagtaatggttttgatggctttgatgttccagagtcactgacatcctcacctaaggatctgtaagagagttccttcaactcggataaaacatgtttcaccactgctgtttctatgtcacttgaatccctggttttctcatgcatattgttcagtagttttagaccatccactttcccacttttagaaatgctggccaaaggagagcctttggtatcagaagagcagcatttcaaactgcactcctcatttataactgggggttctgccataactggattttctttgtgtttgcactttatacttcggaacttgggctgtttgcttttcgaatgtaatagagcttgatttgctgccccaccctttattaacgagttctcactggatatgcttgatgacaggttgaattttggagagagagcatcatttgtaaaatctgactggggtttgtgaacaagagtagatgccttcagatcagagagattaacctgagacgtctcggttccaggctctgcactcttagtacaacccattaagtggtctgtatgtgagttactaatgagaggcttctgttttgcttttaccctagtgtttgtggcagcaaacctagaatactttatcttttcatttttctgcatagataacatgttctctgttctatcgaaagcatctggaatttcaaggacactgttatcagactctgagctgtgttctatgggatccaggtcactgcttccatcatcagaagtggtacagatactaatggaatcacttcgcttttcctcatcacctgctccaatatagcagagcttcacttttgaaccacacaccaggcttcgttggggtttattcttctctcgagaacactttgagatcaaagcaccctcaggcaagcccaataaagagtcaccatttgaagtctcaaattctttctttgcagtgttttttccacaggaagaaaacagaaaacttcctggggcagtgttggaccctgtgaggctatttgctatcctggaaagttcattagaggcctgcgtatcagatatatccccagagataaagtttaggccaaggttctctggaatctttcccctccgttcatctttatgtgcttcaaattgtatgtggccctttttcacactagtcctttttggattatcagagctctttctggctcgagatttagcgcaaggcttttccttctcatctgcagaatgttcagaatcaaaagccagtgatttcaaacagccattaagcaacaggtcatgttctgactcaggatcatttgtgcagtcttcaaatggcatatcttcttcactgtccaacttgattgaaccaggaatacattttcggttctttgaccccttgggaacatcatactgttctgcaagtccaacactggcttcccatttactcaaaattttctgaggaaccttatgcctatatcctttttctttctgtttccctcttctcctaaggacaggtagctcttcgaattgatgtctgccttcaaacatgacgattgcttttccagccacccaggctctctcagaaggatctccaaaagcctccacgtagtactgccgatagggcctccggttggaaactttcatttttgaatgtgtgttaatcaacggatcagaacaaatcctgcagggccaccatgggcgtctcttgaattttgcccagatgagatctccaacttcatacttcagtggcgtagactttttcttaggttgacaaaatggcaattcctgtgaagtagatgatgatgaagttccaggtaattctagcatgtttcctaatgtactggtactggaatctggatcatcctgaaaagataaatttattgagtttaattgctcttctattgtaatgtttgtgtctcctagtgaaaagggggctgggagaagggctgctttttcattgctgccgtccacttcatttctttgcttatttttctgtgtttcagtctgaggagctaatggcaagaatggcgatttgactgcaccgtgtctactctctggtgtgctgtcttgttcacttcccatggccacttttacaccattctctgatttagtctcataattgcaggtggcattggtctgagtttcctcaaagatctcctctatactctcatcctctgtgactggctgttctgggtccatttcagaatctacatctgcatcgtccacacaagtaaaattctcaaagtgcagaaagccattcttgatagtctttgttacttttacctggagttcaggggagttattacaagagggttcctgtttcatagcaagtgctgtaggaccaccaggactcaaggaagtgcaaacaattggcgtctgagctcttgaatcacttttttcagggtcttgaaaggattctgatccatcagcagacccatttaaatactctacattgatcatggaggccaaatcctgtagtctccgcagtggaatgtaacaagatggagaatcttgtccataagcattttgggatgttccactgacagtcgataactgcatagtacacccattaagtggctcagaaaaattggattgaccattaccgaaagggctgtccttgtcttcaggggcatctaaattcactggattggaaaagggcagcagacaatttcttctgggtagttcacaggtctgatccatcctgggccggcatcaacctgaggggaggcggaggccgaggtgttcgcaggcggccggcggggcacgggccgcgccgggaggaagttcgcggcagcccggccagctaggcctgagcccggctg

SEQ ID NO: 19171 - RNA, 12070 nt, Homo sapiens
  source 1..12070: mol_type = other RNA
tgtcttctctcctcccaaacaggaacccgggtttcttgagctgccagtccctcaacccttggcagtgcttatttataccgtgaaattagcaccatcattacattttattgtgtgtgtgtacaaaacaatgatctattcttatttcaatttacactatagcagcctctggccctgttgcactggccctaggaagctcagctgagaactaactggccatagccaatgacaggctcccacagcaactaccaagcagtgacttggaatgtctacacatggaactgctcaaatgaaactcagcaagaaaggggctggaggcagctccttctctgccatgatctgagagaggttaggacactgggctcctctaacctggctgataaaccccaagaggatgacagtatcatttaaaaaaccttagtaaaatccaccttatagggactaagggtaaaacctatccaagtttcatgctgtcctcattactccctatgggggaatctgtcaggactaaactttctgccattctgttctcatgaggcaacattagaattacaacctgggagtccggctccagtgagcagacagtgccgagcctgggaagggatcaacagggtgtttcatgccctgaccatagtgtggggtgaaggatgtaaagaataaaataactattttcatcaatgctaaagatttggttcagaagagggtcaacacagtgatttaagtcatctcaaactcagtaacagggtaaagcagacatttaaaaatgaggatgtttctgtatcaatgacagctattttgctattagactgggttggctccagcaagataagcaaatgaggctttgaatgtaaatttcaacatttttcataatctttttctgacttagcagggctagatgtattggctttctagctacccatggagaatttcaacttttgccttgtccctggaaaaggcctcctggggagctggctccaaggcaaacactcttgagatctcaatttccaagcacatacccaaataccaccctgcgttaaggaccagaagttttctaagatgaaagatttccttttcactccaattcacatccctttggaaaaggggtcttattacaaacttcaggggacgtcccacagggctggcaaggccactccctccccaccttcctccaagagtcacatttcccaacagttgttgtgactctgcttctaattggatagtgactgctttcatgattttaaccatctagtatcacatgctgctactggtgggcccaatagctcaaatttctagtttccagtggttttctagttcccattcaatggcccttgaaggaagcccagatgtccatccattcagatgaagaactgctccccaaaatggctcagaagctgttttcccaggcaggtctggaacgaagcctccaatgaatggcggagaatggaaagaaccaaaataaaaccacaaagcagccaatcatggcccctttccctcactccctcctgtcctgtgagacatctagactgctgtcaagttgattacctaccaaagcctactttagagaagctactttagaatcaaacttctccacggaaaatttttacatggcctgcacgccctccccccgccccccccaaattcacagtttatttcatgaaacaaagagctacggtaatttaacacacaacatagtgaaaggagactctgacagtgcagtgcagatacctttttctgatcacaactacagatgactggagagaaaagggcacaggactggcaccaagcaaaccctactcatatgacctaaaagattagggaaagggacctactagctgcagttatatatttattattctcacacatgataaatacttaatataatgaactttaatgttctcggtgaatttctttaaaaatatctttttcatggtttaaaattcttttaaaagaaaataagatgctttacgttttctcttccttttgaacaaagagcttttcctctttgatgatgtgggaagagagagaggatgaaaggggagaactaggcaggtggaattcacagaggagattccgaggtctcagtgaaatgcagggataggcccctaaactcaggacagccctgcccagcctcgtccctctgcctgagttcaagtgtctcaacctcagagacagactttgggaaataaaagcagattctatttttaatctttagataaagcgcaaatgcttctataataactactgttccctccgtggaattgatgggagtaacctcaataagaacttgaggaaattgggaccaaatacagaatcctattgagagcgtgaaagccataactaagagataatggccaggagacgttagggccggggatggcctgctggctaagttggcaaagcagagaggtaaacatgttggtctaaggacaaaggaggggtagacaagtgggaggaaactagccaaacagcacttcctgttggcagtctgtgagctgggtgaatggtagggcagggtagcaccaacagatttcccagcccttgggccccagctcagggcagcagtaacagataatcagcagttaataggagtcatctcttagcctggacgttgctctaaacaccacctcttgccagtcttcagggaagggttctggcttgcctttgagctaagtcagcaggcaggtgctctcaatacagagcacagcaattctcagggaggcgaagaagaggactccctccactcaggagggaaaaggaatggggaaaagaaatttcccatcaggatctggtactcttcctgaagctggtgtgtctagctcagagcttgccagagattccctatgtccactgcccgaggctctgaaatctgaaagcacctgagtgttttagggaaatagggatggggtggattcatgtacaaagagaaaaataggtagaaacaaaagcaaagaaagagaagcttgccaaatgccttcttccactgctggaaatctacattcgcacagagcccgactgcccctgaccacctgctcctccaaggactgatcttgagactctgcacagcccagacaaaagcagcagcggcgaccccacagccaacagccttgctggcctcaatgcagcacccttgcatctatagaggagacctctgtgagtgtgcgcgcatgcacacgcacccatgcacaccgcagccaagagacacttcctcaacacaaccacttctggtgccacaaaggacatttcaaaatgagtctaaagccccagggcccctcagaacttcctgttacttcctggtcaaaggttcctgaaagccttggaatccaggctcacagggatgaggcctgtatctctcatcagtgactagcacccggcctagaacacgtgaatgctcaggaaatcgccactgatttgaaagaacaccatttcctcccaagggttcctaggtgccctcaatggggctctgtctggttggggaaatcgctttgagagcccctataccttccaacctgaccagcggaattgaattccatacttgactccagagtggactttttatttcacgatgaccatgtggaaaagttgggggaaagagacccaagtctgtctgtctccttggttggggcccactggattttcatacatggttcacacaaccataagcccccactggctaatgtcacaagagttctgagtgttgggatatgaggaaagaataacagtgggaaagtgttcggggcagatgtgtttttttttaagggggaaagaaagaaaagatttcccctccccaaatggtaccctgggggcagcttgtttgttcatgtgacattgattggtactacttctgttctgattctgcacacttgtgactggaaggagcctggttaagagctggaagtgtattttgctctggtttggggtcttgccctcttccaagagaccagcaagtctgtgccaatgtctgtgtgctcccagcagaccagcaagactgtgccagtgtctgtccagccactatgggccagagccctgcccgtgatgaggcttttcccagggcccagggactttgctctgtggttaccaacttcttttcttcagtggggagggaggctggggccttcccgagagacctaaaagattgcccactcttggcggcaagtgcaggtagttgctggcctccgaccatctgcttcgcctgcttcaccaggcccggggattggctaagaggccctggggtctgctcagcccctgcagaagctcttcctgaggcctgagttgttggctcatataaaaaggccttggcaggaggctgagaaagaagtctggcctgggtgagtgatttaacagcttgccaggggtcctctgaaggggctgctgctttcccagatgtctgaagaggatctgacacacagcctttctcaacagctctcggcatatgccccagacctttgctggcaggccatgaacttgactccaacactggcatcttctcatcagcctgtggtgtgacctgatgaggtgaagctgcccgctccttctggcgaggagttaggtctatgagatccatcaccaaagcagctctattttttgactgagtattctggtccacaggcctcagtgctttttctttagctacaagggtctggaccacagctgatagtactttctcaggaggtgggagtctctgggacaaagaggcatggggtttgtcagtaggcctgtctgaagtctggggtttgggactgctagtaatgagcagtctgtctggcggcggaagtctcaggccagtgggaactgaggttttctccagtgactggggccttgggctggcagcacctatggatttatccagccttgggtcagccgtccccagaggtctttccagtggttgggacctgactgagggtgaggagcttgggctggtcactggagagggtttgtcgcttagctggggtcttggtcctgccactgctggtggcctgtccagtggcctctggctggaaaccaaggattgggatttggtccctgacccagcgaggtctctgaccttatctaaaggctggggcctggagtcagttctctcaagaggtctttcaggtagcaatggcctctgacaagtccctgccagagcttttttggagagcgacagcatctggttggtgtcagcaggaggtttatctgacattttgggtgcctgagcagccattcctgttgattgctctgccaggtgagtgcttggccctggaggcagcggtactgggggaggcacatactcacggatctccccaggttccagaggattgggcccacaggggtcatgctcagtacaagacagacgcccatccagtttggaaatgaaaagcatcccttctcgatgctgcttacaaaaggagctggggcacatctcacagaaggaggctgcttccttcccgcagatgtcacactgatgccacggacattcccatttccctgctggtcgcttggtcagattgagacagtctgcgtggtaaacttttgggcagcctggtttcttgcaggagacgagctggccagcatccccacaactaaaacactcatcttctcgctcctttgtgatttcaccctgggtcctgcgctttccctgttgcttcttcttgaatttctttgacttttcttccgtggcaatgggttgattctttggccttacacccaagaagccactgcagttcggggctccacatttgcaaacagtctttccattcccaagacattctaggttgtagttgaaggtaagttcagtgcctgctttaatgtcacttagtgcaaaaaggcctacacgggtatctccattcacagaccacttctgtgtttcacagttgggctggcagcaatgattcatgaaccgagcatagtttcctttgggaccagcatcaatgattcggtctttgtctagggtgagcatatagaaattagtgatatcatgttcttgagcatagcgaattcgagctctgcattcttcttcatctataagctcacccacatactcattcacaaattcaccctttttaatatctgtttttgtccgtagaccccaaccccgctgtaatgtgcggaaaatttcaacctctggatattggcgcttggaaaagcactggttttgacagcgccctccggcaggacacactgtggggtggcactcatagagcagcatgcggttgatgcattcagagtctatcccacaggggttctcatcagtagctttacagttgcaacggggtatttcagataagtctgcagtgaagatctgtaccctgccaataggacggtttacctttatatgtttataaggtggtggcttcttgtcattctttcggtcttcctgcagctgtcttagctctttttgggcctttaattcctcaaaccttgctgcagcttcctgaagagcttttttatatgtcccatccactcctttgcccatcttatccttgctgctcacgtcaccctccatgtaagggaagactcgggcctggtgagtccacaaatagtcattagatccaaaaaagaggactgggaactctcccacatcatgtctcatcttatcaatgttggaaggaacagctcgaggatggcagatctcagctggccaccacctgtatcgtccaacttttacccagacaatctccctgtagtgtggctttttgcctgctttacagtcattgcaataccagtttccttcagggatatcaatgttcaggcattcacgatgaaaagcagcagggcaagaatcacagcacagaaggctgcctccttctgagcacacaaagcaccagctaacattaacatgctcatgatttcggcagccccgcctaggggtaaagtgattagggcagatgatactattagatgcaaggatctttgacccagcagccaggcaaaagtcattggcgtggtatgccacaggacagcggacacagcgcatcaaccgacctttagatgcagaaacattggctggattagcagcatgacaggttatacagatgtggagggagcaccggaagcccttgttctgcataacagtgggtgggtacttctggacacactcttcatggtaaaactttccacacaagggtagaaggcaccttttaacatcttccccactctgcttacatacaaaacaggtatggattcctgtgcgacattcattgcagataaattttcctcttggcatctcagtcaatccaaggcactccaggtggaaagccccacagcactgagcctcacataacagcagctcacccaatttttcacaattctgacagacattctccttgagtgcagctcctccaccgcgttcaccctgcatttttttagaggcaggcatcccgggatcgtgttctacaccttcctcaacagtctccttggggcttgtggccgtcctgtgaggcattagttctccctctgagcctggaatctcttttgacgagtcatcatttttcacttttttacactgcatcttggctgcagcatgcctctgtcgttttcgcttccttggcttgtcaaatatcttggtagtgcctccaccaaaatcttttgaataagatgtggcacaagattcagttatgccattctccaggtgaccagcttcatagcactttttagaaaggccaaggtcccccttcttgggcataaatccagggtctaaatcattggattcaagaagtttcttagttggttttctttgacgtttactttcataatttcctggcgttttaactagcaattcctcagactcaagggcaggccgtggagagacttccggagccacaggcacagacaaggtcagctgcggcaactcagcatgtccacctccaagttctgactgagccaaggggccctccaaaaacggagcctccctttcaagaactggaggctcttctttggttgaaatcaaagaattctcgtccacctgcttgttctgagcactagatcgacctcgggctagaaggctttcctcttcacagcgggaacttaccttgtgcacctgctcctgtaccttcttttgttttttcttaggagcaaatatctgatcatattcttctgtatattccaaaagccacttgcttggcttcctaaggcgtttcttctctgaccgcacagctggttcagggagctcagcctgtggtgtcaaactgggaattcctggctccttttccatgtcaccaatgctggcactggatttatcacaaacatttaaccgtggcccagctgaatctaagcagtcagcatgattttgctctgtcagtggttcctcaagtatgcttgctgaaggagttctatgctctggaaactcatcccgcccctcctgcacagggtcactaggaagtaagaccctaaaggcacactcagagttttctttctctttaaatctgttcatgcgcttacgaggtttagtgcgcctttggtttaaacgctgccaccgctttttaggcaccacttgatttacaccattgagttcatcattctcactgttcattacagagtccagctctgggccttttccgttttcaaaagagagtcctttttcagaaattttaccaggatcagattgcttaaccttgctatcgaaatgcacatcagaaaaatggtcaccatcttcacttgttaagtggcccattatctgaaggggatcctctttactaggatcttctgccccacctctcaatgaacctccacgttctcggtctccctgcagtacagcatcaagagtcacacttggaagctgattcagttttcttttgcgctcggtctttaaggctttacggttcactgtgttctttaccatttgggctgaaaaagcatctcgcaatttggatgaaggctttgatcgtccacagttgcgcctagtaacacagtctgaacgacttttaccagaagcagggaggtctctcttgtcggacagtaagccaggtagggaagcagacaactcgccagataatgcagagtcacccccactagggctaggattggcggagttctgagtgccatctccctttttctctgaattgtgtgtggagcctcctgaaaccaaaaccttagagactcctacaggactattagtagaacagtccccacgaccaggactccggtaagagaccaggttttgagcagtcatcaaccgctgctccttcgtcttactatcatgcatatctttcaacatcattagcaatgtactgaatttgtagtctggttcaataggtatgtgattctgactagaagcagaagagaaaagtaatggttttgatggctttgatgttccagagtcactgacatcctcacctaaggatctgtaagagagttccttcaactcggataaaacatgtttcaccactgctgtttctatgtcacttgaatccctggttttctcatgcatattgttcagtagttttagaccatccactttcccacttttagaaatgctggccaaaggagagcctttggtatcagaagagcagcatttcaaactgcactcctcatttataactgggggttctgccataactggattttctttgtgtttgcactttatacttcggaacttgggctgtttgcttttcgaatgtaatagagcttgatttgctgccccaccctttattaacgagttctcactggatatgcttgatgacaggttgaattttggagagagagcatcatttgtaaaatctgactggggtttgtgaacaagagtagatgccttcagatcagagagattaacctgagacgtctcggttccaggctctgcactcttagtacaacccattaagtggtctgtatgtgagttactaatgagaggcttctgttttgcttttaccctagtgtttgtggcagcaaacctagaatactttatcttttcatttttctgcatagataacatgttctctgttctatcgaaagcatctggaatttcaaggacactgttatcagactctgagctgtgttctatgggatccaggtcactgcttccatcatcagaagtggtacagatactaatggaatcacttcgcttttcctcatcacctgctccaatatagcagagcttcacttttgaaccacacaccaggcttcgttggggtttattcttctctcgagaacactttgagatcaaagcaccctcaggcaagcccaataaagagtcaccatttgaagtctcaaattctttctttgcagtgttttttccacaggaagaaaacagaaaacttcctggggcagtgttggaccctgtgaggctatttgctatcctggaaagttcattagaggcctgcgtatcagatatatccccagagataaagtttaggccaaggttctctggaatctttcccctccgttcatctttatgtgcttcaaattgtatgtggccctttttcacactagtcctttttggattatcagagctctttctggctcgagatttagcgcaaggcttttccttctcatctgcagaatgttcagaatcaaaagccagtgatttcaaacagccattaagcaacaggtcatgttctgactcaggatcatttgtgcagtcttcaaatggcatatcttcttcactgtccaacttgattgaaccaggaatacattttcggttctttgaccccttgggaacatcatactgttctgcaagtccaacactggcttcccatttactcaaaattttctgaggaaccttatgcctatatcctttttctttctgtttccctcttctcctaaggacaggtagctcttcgaattgatgtctgccttcaaacatgacgattgcttttccagccacccaggctctctcagaaggatctccaaaagcctccacgtagtactgccgatagggcctccggttggaaactttcatttttgaatgtgtgttaatcaacggatcagaacaaatcctgcagggccaccatgggcgtctcttgaattttgcccagatgagatctccaacttcatacttcagtggcgtagactttttcttaggttgacaaaatggcaattcctgtgaagtagatgatgatgaagttccaggtaattctagcatgtttcctaatgtactggtactggaatctggatcatcctgaaaagataaatttattgagtttaattgctcttctattgtaatgtttgtgtctcctagtgaaaagggggctgggagaagggctgctttttcattgctgccgtccacttcatttctttgcttatttttctgtgtttcagtctgaggagctaatggcaagaatggcgatttgactgcaccgtgtctactctctggtgtgctgtcttgttcacttcccatggccacttttacaccattctctgatttagtctcataattgcaggtggcattggtctgagtttcctcaaagatctcctctatactctcatcctctgtgactggctgttctgggtccatttcagaatctacatctgcatcgtccacacaagtaaaattctcaaagtgcagaaagccattcttgatagtctttgttacttttacctggagttcaggggagttattacaagagggttcctgtttcatagcaagtgctgtaggaccaccaggactcaaggaagtgcaaacaattggcgtctgagctcttgaatcacttttttcagggtcttgaaaggattctgatccatcagcagacccatttaaatactctacattgatcatggaggccaaatcctgtagtctccgcagtggaatgtaacaagatggagaatcttgtccataagcattttgggatgttccactgacagtcgataactgcatagtacacccattaagtggctcagaaaaattggattgaccattaccgaaagggctgtccttgtcttcaggggcatctaaattcactggattggaaaagggcagcagacaatttcttctgggtagttcacaggtctgatccatcctgggccggcatcaacctgggggcttgggctggggtcttcgaggcctcaggccccgagcagacgcggccgcaggcgaaccccctacccggccgcaccccaaacccacaccaccaccaccaccaccaccacagaccaagctgagcag

SEQ ID NO: 19172 - RNA, 11999 nt, Homo sapiens
  source 1..11999: mol_type = other RNA
tgtcttctctcctcccaaacaggaacccgggtttcttgagctgccagtccctcaacccttggcagtgcttatttataccgtgaaattagcaccatcattacattttattgtgtgtgtgtacaaaacaatgatctattcttatttcaatttacactatagcagcctctggccctgttgcactggccctaggaagctcagctgagaactaactggccatagccaatgacaggctcccacagcaactaccaagcagtgacttggaatgtctacacatggaactgctcaaatgaaactcagcaagaaaggggctggaggcagctccttctctgccatgatctgagagaggttaggacactgggctcctctaacctggctgataaaccccaagaggatgacagtatcatttaaaaaaccttagtaaaatccaccttatagggactaagggtaaaacctatccaagtttcatgctgtcctcattactccctatgggggaatctgtcaggactaaactttctgccattctgttctcatgaggcaacattagaattacaacctgggagtccggctccagtgagcagacagtgccgagcctgggaagggatcaacagggtgtttcatgccctgaccatagtgtggggtgaaggatgtaaagaataaaataactattttcatcaatgctaaagatttggttcagaagagggtcaacacagtgatttaagtcatctcaaactcagtaacagggtaaagcagacatttaaaaatgaggatgtttctgtatcaatgacagctattttgctattagactgggttggctccagcaagataagcaaatgaggctttgaatgtaaatttcaacatttttcataatctttttctgacttagcagggctagatgtattggctttctagctacccatggagaatttcaacttttgccttgtccctggaaaaggcctcctggggagctggctccaaggcaaacactcttgagatctcaatttccaagcacatacccaaataccaccctgcgttaaggaccagaagttttctaagatgaaagatttccttttcactccaattcacatccctttggaaaaggggtcttattacaaacttcaggggacgtcccacagggctggcaaggccactccctccccaccttcctccaagagtcacatttcccaacagttgttgtgactctgcttctaattggatagtgactgctttcatgattttaaccatctagtatcacatgctgctactggtgggcccaatagctcaaatttctagtttccagtggttttctagttcccattcaatggcccttgaaggaagcccagatgtccatccattcagatgaagaactgctccccaaaatggctcagaagctgttttcccaggcaggtctggaacgaagcctccaatgaatggcggagaatggaaagaaccaaaataaaaccacaaagcagccaatcatggcccctttccctcactccctcctgtcctgtgagacatctagactgctgtcaagttgattacctaccaaagcctactttagagaagctactttagaatcaaacttctccacggaaaatttttacatggcctgcacgccctccccccgccccccccaaattcacagtttatttcatgaaacaaagagctacggtaatttaacacacaacatagtgaaaggagactctgacagtgcagtgcagatacctttttctgatcacaactacagatgactggagagaaaagggcacaggactggcaccaagcaaaccctactcatatgacctaaaagattagggaaagggacctactagctgcagttatatatttattattctcacacatgataaatacttaatataatgaactttaatgttctcggtgaatttctttaaaaatatctttttcatggtttaaaattcttttaaaagaaaataagatgctttacgttttctcttccttttgaacaaagagcttttcctctttgatgatgtgggaagagagagaggatgaaaggggagaactaggcaggtggaattcacagaggagattccgaggtctcagtgaaatgcagggataggcccctaaactcaggacagccctgcccagcctcgtccctctgcctgagttcaagtgtctcaacctcagagacagactttgggaaataaaagcagattctatttttaatctttagataaagcgcaaatgcttctataataactactgttccctccgtggaattgatgggagtaacctcaataagaacttgaggaaattgggaccaaatacagaatcctattgagagcgtgaaagccataactaagagataatggccaggagacgttagggccggggatggcctgctggctaagttggcaaagcagagaggtaaacatgttggtctaaggacaaaggaggggtagacaagtgggaggaaactagccaaacagcacttcctgttggcagtctgtgagctgggtgaatggtagggcagggtagcaccaacagatttcccagcccttgggccccagctcagggcagcagtaacagataatcagcagttaataggagtcatctcttagcctggacgttgctctaaacaccacctcttgccagtcttcagggaagggttctggcttgcctttgagctaagtcagcaggcaggtgctctcaatacagagcacagcaattctcagggaggcgaagaagaggactccctccactcaggagggaaaaggaatggggaaaagaaatttcccatcaggatctggtactcttcctgaagctggtgtgtctagctcagagcttgccagagattccctatgtccactgcccgaggctctgaaatctgaaagcacctgagtgttttagggaaatagggatggggtggattcatgtacaaagagaaaaataggtagaaacaaaagcaaagaaagagaagcttgccaaatgccttcttccactgctggaaatctacattcgcacagagcccgactgcccctgaccacctgctcctccaaggactgatcttgagactctgcacagcccagacaaaagcagcagcggcgaccccacagccaacagccttgctggcctcaatgcagcacccttgcatctatagaggagacctctgtgagtgtgcgcgcatgcacacgcacccatgcacaccgcagccaagagacacttcctcaacacaaccacttctggtgccacaaaggacatttcaaaatgagtctaaagccccagggcccctcagaacttcctgttacttcctggtcaaaggttcctgaaagccttggaatccaggctcacagggatgaggcctgtatctctcatcagtgactagcacccggcctagaacacgtgaatgctcaggaaatcgccactgatttgaaagaacaccatttcctcccaagggttcctaggtgccctcaatggggctctgtctggttggggaaatcgctttgagagcccctataccttccaacctgaccagcggaattgaattccatacttgactccagagtggactttttatttcacgatgaccatgtggaaaagttgggggaaagagacccaagtctgtctgtctccttggttggggcccactggattttcatacatggttcacacaaccataagcccccactggctaatgtcacaagagttctgagtgttgggatatgaggaaagaataacagtgggaaagtgttcggggcagatgtgtttttttttaagggggaaagaaagaaaagatttcccctccccaaatggtaccctgggggcagcttgtttgttcatgtgacattgattggtactacttctgttctgattctgcacacttgtgactggaaggagcctggttaagagctggaagtgtattttgctctggtttggggtcttgccctcttccaagagaccagcaagtctgtgccaatgtctgtgtgctcccagcagaccagcaagactgtgccagtgtctgtccagccactatgggccagagccctgcccgtgatgaggcttttcccagggcccagggactttgctctgtggttaccaacttcttttcttcagtggggagggaggctggggccttcccgagagacctaaaagattgcccactcttggcggcaagtgcaggtagttgctggcctccgaccatctgcttcgcctgcttcaccaggcccggggattggctaagaggccctggggtctgctcagcccctgcagaagctcttcctgaggcctgagttgttggctcatataaaaaggccttggcaggaggctgagaaagaagtctggcctgggtgagtgatttaacagcttgccaggggtcctctgaaggggctgctgctttcccagatgtctgaagaggatctgacacacagcctttctcaacagctctcggcatatgccccagacctttgctggcaggccatgaacttgactccaacactggcatcttctcatcagcctgtggtgtgacctgatgaggtgaagctgcccgctccttctggcgaggagttaggtctatgagatccatcaccaaagcagctctattttttgactgagtattctggtccacaggcctcagtgctttttctttagctacaagggtctggaccacagctgatagtactttctcaggaggtgggagtctctgggacaaagaggcatggggtttgtcagtaggcctgtctgaagtctggggtttgggactgctagtaatgagcagtctgtctggcggcggaagtctcaggccagtgggaactgaggttttctccagtgactggggccttgggctggcagcacctatggatttatccagccttgggtcagccgtccccagaggtctttccagtggttgggacctgactgagggtgaggagcttgggctggtcactggagagggtttgtcgcttagctggggtcttggtcctgccactgctggtggcctgtccagtggcctctggctggaaaccaaggattgggatttggtccctgacccagcgaggtctctgaccttatctaaaggctggggcctggagtcagttctctcaagaggtctttcaggtagcaatggcctctgacaagtccctgccagagcttttttggagagcgacagcatctggttggtgtcagcaggaggtttatctgacattttgggtgcctgagcagccattcctgttgattgctctgccaggtgagtgcttggccctggaggcagcggtactgggggaggcacatactcacggatctccccaggttccagaggattgggcccacaggggtcatgctcagtacaagacagacgcccatccagtttggaaatgaaaagcatcccttctcgatgctgcttacaaaaggagctggggcacatctcacagaaggaggctgcttccttcccgcagatgtcacactgatgccacggacattcccatttccctgctggtcgcttggtcagattgagacagtctgcgtggtaaacttttgggcagcctggtttcttgcaggagacgagctggccagcatccccacaactaaaacactcatcttctcgctcctttgtgatttcaccctgggtcctgcgctttccctgttgcttcttcttgaatttctttgacttttcttccgtggcaatgggttgattctttggccttacacccaagaagccactgcagttcggggctccacatttgcaaacagtctttccattcccaagacattctaggttgtagttgaaggtaagttcagtgcctgctttaatgtcacttagtgcaaaaaggcctacacgggtatctccattcacagaccacttctgtgtttcacagttgggctggcagcaatgattcatgaaccgagcatagtttcctttgggaccagcatcaatgattcggtctttgtctagggtgagcatatagaaattagtgatatcatgttcttgagcatagcgaattcgagctctgcattcttcttcatctataagctcacccacatactcattcacaaattcaccctttttaatatctgtttttgtccgtagaccccaaccccgctgtaatgtgcggaaaatttcaacctctggatattggcgcttggaaaagcactggttttgacagcgccctccggcaggacacactgtggggtggcactcatagagcagcatgcggttgatgcattcagagtctatcccacaggggttctcatcagtagctttacagttgcaacggggtatttcagataagtctgcagtgaagatctgtaccctgccaataggacggtttacctttatatgtttataaggtggtggcttcttgtcattctttcggtcttcctgcagctgtcttagctctttttgggcctttaattcctcaaaccttgctgcagcttcctgaagagcttttttatatgtcccatccactcctttgcccatcttatccttgctgctcacgtcaccctccatgtaagggaagactcgggcctggtgagtccacaaatagtcattagatccaaaaaagaggactgggaactctcccacatcatgtctcatcttatcaatgttggaaggaacagctcgaggatggcagatctcagctggccaccacctgtatcgtccaacttttacccagacaatctccctgtagtgtggctttttgcctgctttacagtcattgcaataccagtttccttcagggatatcaatgttcaggcattcacgatgaaaagcagcagggcaagaatcacagcacagaaggctgcctccttctgagcacacaaagcaccagctaacattaacatgctcatgatttcggcagccccgcctaggggtaaagtgattagggcagatgatactattagatgcaaggatctttgacccagcagccaggcaaaagtcattggcgtggtatgccacaggacagcggacacagcgcatcaaccgacctttagatgcagaaacattggctggattagcagcatgacaggttatacagatgtggagggagcaccggaagcccttgttctgcataacagtgggtgggtacttctggacacactcttcatggtaaaactttccacacaagggtagaaggcaccttttaacatcttccccactctgcttacatacaaaacaggtatggattcctgtgcgacattcattgcagataaattttcctcttggcatctcagtcaatccaaggcactccaggtggaaagccccacagcactgagcctcacataacagcagctcacccaatttttcacaattctgacagacattctccttgagtgcagctcctccaccgcgttcaccctgcatttttttagaggcaggcatcccgggatcgtgttctacaccttcctcaacagtctccttggggcttgtggccgtcctgtgaggcattagttctccctctgagcctggaatctcttttgacgagtcatcatttttcacttttttacactgcatcttggctgcagcatgcctctgtcgttttcgcttccttggcttgtcaaatatcttggtagtgcctccaccaaaatcttttgaataagatgtggcacaagattcagttatgccattctccaggtgaccagcttcatagcactttttagaaaggccaaggtcccccttcttgggcataaatccagggtctaaatcattggattcaagaagtttcttagttggttttctttgacgtttactttcataatttcctggcgttttaactagcaattcctcagactcaagggcaggccgtggagagacttccggagccacaggcacagacaaggtcagctgcggcaactcagcatgtccacctccaagttctgactgagccaaggggccctccaaaaacggagcctccctttcaagaactggaggctcttctttggttgaaatcaaagaattctcgtccacctgcttgttctgagcactagatcgacctcgggctagaaggctttcctcttcacagcgggaacttaccttgtgcacctgctcctgtaccttcttttgttttttcttaggagcaaatatctgatcatattcttctgtatattccaaaagccacttgcttggcttcctaaggcgtttcttctctgaccgcacagctggttcagggagctcagcctgtggtgtcaaactgggaattcctggctccttttccatgtcaccaatgctggcactggatttatcacaaacatttaaccgtggcccagctgaatctaagcagtcagcatgattttgctctgtcagtggttcctcaagtatgcttgctgaaggagttctatgctctggaaactcatcccgcccctcctgcacagggtcactaggaagtaagaccctaaaggcacactcagagttttctttctctttaaatctgttcatgcgcttacgaggtttagtgcgcctttggtttaaacgctgccaccgctttttaggcaccacttgatttacaccattgagttcatcattctcactgttcattacagagtccagctctgggccttttccgttttcaaaagagagtcctttttcagaaattttaccaggatcagattgcttaaccttgctatcgaaatgcacatcagaaaaatggtcaccatcttcacttgttaagtggcccattatctgaaggggatcctctttactaggatcttctgccccacctctcaatgaacctccacgttctcggtctccctgcagtacagcatcaagagtcacacttggaagctgattcagttttcttttgcgctcggtctttaaggctttacggttcactgtgttctttaccatttgggctgaaaaagcatctcgcaatttggatgaaggctttgatcgtccacagttgcgcctagtaacacagtctgaacgacttttaccagaagcagggaggtctctcttgtcggacagtaagccaggtagggaagcagacaactcgccagataatgcagagtcacccccactagggctaggattggcggagttctgagtgccatctccctttttctctgaattgtgtgtggagcctcctgaaaccaaaaccttagagactcctacaggactattagtagaacagtccccacgaccaggactccggtaagagaccaggttttgagcagtcatcaaccgctgctccttcgtcttactatcatgcatatctttcaacatcattagcaatgtactgaatttgtagtctggttcaataggtatgtgattctgactagaagcagaagagaaaagtaatggttttgatggctttgatgttccagagtcactgacatcctcacctaaggatctgtaagagagttccttcaactcggataaaacatgtttcaccactgctgtttctatgtcacttgaatccctggttttctcatgcatattgttcagtagttttagaccatccactttcccacttttagaaatgctggccaaaggagagcctttggtatcagaagagcagcatttcaaactgcactcctcatttataactgggggttctgccataactggattttctttgtgtttgcactttatacttcggaacttgggctgtttgcttttcgaatgtaatagagcttgatttgctgccccaccctttattaacgagttctcactggatatgcttgatgacaggttgaattttggagagagagcatcatttgtaaaatctgactggggtttgtgaacaagagtagatgccttcagatcagagagattaacctgagacgtctcggttccaggctctgcactcttagtacaacccattaagtggtctgtatgtgagttactaatgagaggcttctgttttgcttttaccctagtgtttgtggcagcaaacctagaatactttatcttttcatttttctgcatagataacatgttctctgttctatcgaaagcatctggaatttcaaggacactgttatcagactctgagctgtgttctatgggatccaggtcactgcttccatcatcagaagtggtacagatactaatggaatcacttcgcttttcctcatcacctgctccaatatagcagagcttcacttttgaaccacacaccaggcttcgttggggtttattcttctctcgagaacactttgagatcaaagcaccctcaggcaagcccaataaagagtcaccatttgaagtctcaaattctttctttgcagtgttttttccacaggaagaaaacagaaaacttcctggggcagtgttggaccctgtgaggctatttgctatcctggaaagttcattagaggcctgcgtatcagatatatccccagagataaagtttaggccaaggttctctggaatctttcccctccgttcatctttatgtgcttcaaattgtatgtggccctttttcacactagtcctttttggattatcagagctctttctggctcgagatttagcgcaaggcttttccttctcatctgcagaatgttcagaatcaaaagccagtgatttcaaacagccattaagcaacaggtcatgttctgactcaggatcatttgtgcagtcttcaaatggcatatcttcttcactgtccaacttgattgaaccaggaatacattttcggttctttgaccccttgggaacatcatactgttctgcaagtccaacactggcttcccatttactcaaaattttctgaggaaccttatgcctatatcctttttctttctgtttccctcttctcctaaggacaggtagctcttcgaattgatgtctgccttcaaacatgacgattgcttttccagccacccaggctctctcagaaggatctccaaaagcctccacgtagtactgccgatagggcctccggttggaaactttcatttttgaatgtgtgttaatcaacggatcagaacaaatcctgcagggccaccatgggcgtctcttgaattttgcccagatgagatctccaacttcatacttcagtggcgtagactttttcttaggttgacaaaatggcaattcctgtgaagtagatgatgatgaagttccaggtaattctagcatgtttcctaatgtactggtactggaatctggatcatcctgaaaagataaatttattgagtttaattgctcttctattgtaatgtttgtgtctcctagtgaaaagggggctgggagaagggctgctttttcattgctgccgtccacttcatttctttgcttatttttctgtgtttcagtctgaggagctaatggcaagaatggcgatttgactgcaccgtgtctactctctggtgtgctgtcttgttcacttcccatggccacttttacaccattctctgatttagtctcataattgcaggtggcattggtctgagtttcctcaaagatctcctctatactctcatcctctgtgactggctgttctgggtccatttcagaatctacatctgcatcgtccacacaagtaaaattctcaaagtgcagaaagccattcttgatagtctttgttacttttacctggagttcaggggagttattacaagagggttcctgtttcatagcaagtgctgtaggaccaccaggactcaaggaagtgcaaacaattggcgtctgagctcttgaatcacttttttcagggtcttgaaaggattctgatccatcagcagacccatttaaatactctacattgatcatggaggccaaatcctgtagtctccgcagtggaatgtaacaagatggagaatcttgtccataagcattttgggatgttccactgacagtcgataactgcatagtacacccattaagtggctcagaaaaattggattgaccattaccgaaagggctgtccttgtcttcaggggcatctaaattcactggattggaaaagggcagcagacaatttcttctgggtagttcacaggtctgatccatcctgggccggcatcaactcttcggggttcagggcgggtgaagtcgggcttgtgagagcgccgcccaatcagcggag

SEQ ID NO: 19173 - RNA, 11711 nt, Homo sapiens
  source 1..11711: mol_type = other RNA
tgtcttctctcctcccaaacaggaacccgggtttcttgagctgccagtccctcaacccttggcagtgcttatttataccgtgaaattagcaccatcattacattttattgtgtgtgtgtacaaaacaatgatctattcttatttcaatttacactatagcagcctctggccctgttgcactggccctaggaagctcagctgagaactaactggccatagccaatgacaggctcccacagcaactaccaagcagtgacttggaatgtctacacatggaactgctcaaatgaaactcagcaagaaaggggctggaggcagctccttctctgccatgatctgagagaggttaggacactgggctcctctaacctggctgataaaccccaagaggatgacagtatcatttaaaaaaccttagtaaaatccaccttatagggactaagggtaaaacctatccaagtttcatgctgtcctcattactccctatgggggaatctgtcaggactaaactttctgccattctgttctcatgaggcaacattagaattacaacctgggagtccggctccagtgagcagacagtgccgagcctgggaagggatcaacagggtgtttcatgccctgaccatagtgtggggtgaaggatgtaaagaataaaataactattttcatcaatgctaaagatttggttcagaagagggtcaacacagtgatttaagtcatctcaaactcagtaacagggtaaagcagacatttaaaaatgaggatgtttctgtatcaatgacagctattttgctattagactgggttggctccagcaagataagcaaatgaggctttgaatgtaaatttcaacatttttcataatctttttctgacttagcagggctagatgtattggctttctagctacccatggagaatttcaacttttgccttgtccctggaaaaggcctcctggggagctggctccaaggcaaacactcttgagatctcaatttccaagcacatacccaaataccaccctgcgttaaggaccagaagttttctaagatgaaagatttccttttcactccaattcacatccctttggaaaaggggtcttattacaaacttcaggggacgtcccacagggctggcaaggccactccctccccaccttcctccaagagtcacatttcccaacagttgttgtgactctgcttctaattggatagtgactgctttcatgattttaaccatctagtatcacatgctgctactggtgggcccaatagctcaaatttctagtttccagtggttttctagttcccattcaatggcccttgaaggaagcccagatgtccatccattcagatgaagaactgctccccaaaatggctcagaagctgttttcccaggcaggtctggaacgaagcctccaatgaatggcggagaatggaaagaaccaaaataaaaccacaaagcagccaatcatggcccctttccctcactccctcctgtcctgtgagacatctagactgctgtcaagttgattacctaccaaagcctactttagagaagctactttagaatcaaacttctccacggaaaatttttacatggcctgcacgccctccccccgccccccccaaattcacagtttatttcatgaaacaaagagctacggtaatttaacacacaacatagtgaaaggagactctgacagtgcagtgcagatacctttttctgatcacaactacagatgactggagagaaaagggcacaggactggcaccaagcaaaccctactcatatgacctaaaagattagggaaagggacctactagctgcagttatatatttattattctcacacatgataaatacttaatataatgaactttaatgttctcggtgaatttctttaaaaatatctttttcatggtttaaaattcttttaaaagaaaataagatgctttacgttttctcttccttttgaacaaagagcttttcctctttgatgatgtgggaagagagagaggatgaaaggggagaactaggcaggtggaattcacagaggagattccgaggtctcagtgaaatgcagggataggcccctaaactcaggacagccctgcccagcctcgtccctctgcctgagttcaagtgtctcaacctcagagacagactttgggaaataaaagcagattctatttttaatctttagataaagcgcaaatgcttctataataactactgttccctccgtggaattgatgggagtaacctcaataagaacttgaggaaattgggaccaaatacagaatcctattgagagcgtgaaagccataactaagagataatggccaggagacgttagggccggggatggcctgctggctaagttggcaaagcagagaggtaaacatgttggtctaaggacaaaggaggggtagacaagtgggaggaaactagccaaacagcacttcctgttggcagtctgtgagctgggtgaatggtagggcagggtagcaccaacagatttcccagcccttgggccccagctcagggcagcagtaacagataatcagcagttaataggagtcatctcttagcctggacgttgctctaaacaccacctcttgccagtcttcagggaagggttctggcttgcctttgagctaagtcagcaggcaggtgctctcaatacagagcacagcaattctcagggaggcgaagaagaggactccctccactcaggagggaaaaggaatggggaaaagaaatttcccatcaggatctggtactcttcctgaagctggtgtgtctagctcagagcttgccagagattccctatgtccactgcccgaggctctgaaatctgaaagcacctgagtgttttagggaaatagggatggggtggattcatgtacaaagagaaaaataggtagaaacaaaagcaaagaaagagaagcttgccaaatgccttcttccactgctggaaatctacattcgcacagagcccgactgcccctgaccacctgctcctccaaggactgatcttgagactctgcacagcccagacaaaagcagcagcggcgaccccacagccaacagccttgctggcctcaatgcagcacccttgcatctatagaggagacctctgtgagtgtgcgcgcatgcacacgcacccatgcacaccgcagccaagagacacttcctcaacacaaccacttctggtgccacaaaggacatttcaaaatgagtctaaagccccagggcccctcagaacttcctgttacttcctggtcaaaggttcctgaaagccttggaatccaggctcacagggatgaggcctgtatctctcatcagtgactagcacccggcctagaacacgtgaatgctcaggaaatcgccactgatttgaaagaacaccatttcctcccaagggttcctaggtgccctcaatggggctctgtctggttggggaaatcgctttgagagcccctataccttccaacctgaccagcggaattgaattccatacttgactccagagtggactttttatttcacgatgaccatgtggaaaagttgggggaaagagacccaagtctgtctgtctccttggttggggcccactggattttcatacatggttcacacaaccataagcccccactggctaatgtcacaagagttctgagtgttgggatatgaggaaagaataacagtgggaaagtgttcggggcagatgtgtttttttttaagggggaaagaaagaaaagatttcccctccccaaatggtaccctgggggcagcttgtttgttcatgtgacattgattggtactacttctgttctgattctgcacacttgtgactggaaggagcctggttaagagctggaagtgtattttgctctggtttggggtcttgccctcttccaagagaccagcaagtctgtgccaatgtctgtgtgctcccagcagaccagcaagactgtgccagtgtctgtccagccactatgggccagagccctgcccgtgatgaggcttttcccagggcccagggactttgctctgtggttaccaacttcttttcttcagtggggagggaggctggggccttcccgagagacctaaaagattgcccactcttggcggcaagtgcaggtagttgctggcctccgaccatctgcttcgcctgcttcaccaggcccggggattggctaagaggccctggggtctgctcagcccctgcagaagctcttcctgaggcctgagttgttggctcatataaaaaggccttggcaggaggctgagaaagaagtctggcctgggtgagtgatttaacagcttgccaggggtcctctgaaggggctgctgctttcccagatgtctgaagaggatctgacacacagcctttctcaacagctctcggcatatgccccagacctttgctggcaggccatgaacttgactccaacactggcatcttctcatcagcctgtggtgtgacctgatgaggtgaagctgcccgctccttctggcgaggagttaggtctatgagatccatcaccaaagcagctctattttttgactgagtattctggtccacaggcctcagtgctttttctttagctacaagggtctggaccacagctgatagtactttctcaggaggtgggagtctctgggacaaagaggcatggggtttgtcagtaggcctgtctgaagtctggggtttgggactgctagtaatgagcagtctgtctggcggcggaagtctcaggccagtgggaactgaggttttctccagtgactggggccttgggctggcagcacctatggatttatccagccttgggtcagccgtccccagaggtctttccagtggttgggacctgactgagggtgaggagcttgggctggtcactggagagggtttgtcgcttagctggggtcttggtcctgccactgctggtggcctgtccagtggcctctggctggaaaccaaggattgggatttggtccctgacccagcgaggtctctgaccttatctaaaggctggggcctggagtcagttctctcaagaggtctttcaggtagcaatggcctctgacaagtccctgccagagcttttttggagagcgacagcatctggttggtgtcagcaggaggtttatctgacattttgggtgcctgagcagccattcctgttgattgctctgccaggtgagtgcttggccctggaggcagcggtactgggggaggcacatactcacggatctccccaggttccagaggattgggcccacaggggtcatgctcagtacaagacagacgcccatccagtttggaaatgaaaagcatcccttctcgatgctgcttacaaaaggagctggggcacatctcacagaaggaggctgcttccttcccgcagatgtcacactgatgccacggacattcccatttccctgctggtcgcttggtcagattgagacagtctgcgtggtaaacttttgggcagcctggtttcttgcaggagacgagctggccagcatccccacaactaaaacactcatcttctcgctcctttgtgatttcaccctgggtcctgcgctttccctgttgcttcttcttgaatttctttgacttttcttccgtggcaatgggttgattctttggccttacacccaagaagccactgcagttcggggctccacatttgcaaacagtctttccattcccaagacattctaggttgtagttgaaggtaagttcagtgcctgctttaatgtcacttagtgcaaaaaggcctacacgggtatctccattcacagaccacttctgtgtttcacagttgggctggcagcaatgattcatgaaccgagcatagtttcctttgggaccagcatcaatgattcggtctttgtctagggtgagcatatagaaattagtgatatcatgttcttgagcatagcgaattcgagctctgcattcttcttcatctataagctcacccacatactcattcacaaattcaccctttttaatatctgtttttgtccgtagaccccaaccccgctgtaatgtgcggaaaatttcaacctctggatattggcgcttggaaaagcactggttttgacagcgccctccggcaggacacactgtggggtggcactcatagagcagcatgcggttgatgcattcagagtctatcccacaggggttctcatcagtagctttacagttgcaacggggtatttcagataagtctgcagtgaagatctgtaccctgccaataggacggtttacctttatatgtttataaggtggtggcttcttgtcattctttcggtcttcctgcagctgtcttagctctttttgggcctttaattcctcaaaccttgctgcagcttcctgaagagcttttttatatgtcccatccactcctttgcccatcttatccttgctgctcacgtcaccctccatgtaagggaagactcgggcctggtgagtccacaaatagtcattagatccaaaaaagaggactgggaactctcccacatcatgtctcatcttatcaatgttggaaggaacagctcgaggatggcagatctcagctggccaccacctgtatcgtccaacttttacccagacaatctccctgtagtgtggctttttgcctgctttacagtcattgcaataccagtttccttcagggatatcaatgttcaggcattcacgatgaaaagcagcagggcaagaatcacagcacagaaggctgcctccttctgagcacacaaagcaccagctaacattaacatgctcatgatttcggcagccccgcctaggggtaaagtgattagggcagatgatactattagatgcaaggatctttgacccagcagccaggcaaaagtcattggcgtggtatgccacaggacagcggacacagcgcatcaaccgacctttagatgcagaaacattggctggattagcagcatgacaggttatacagatgtggagggagcaccggaagcccttgttctgcataacagtgggtgggtacttctggacacactcttcatggtaaaactttccacacaagggtagaaggcaccttttaacatcttccccactctgcttacatacaaaacaggtatggattcctgtgcgacattcattgcagataaattttcctcttggcatctcagtcaatccaaggcactccaggtggaaagccccacagcactgagcctcacataacagcagctcacccaatttttcacaattctgacagacattctccttgagtgcagctcctccaccgcgttcaccctgcatttttttagaggcaggcatcccgggatcgtgttctacaccttcctcaacagtctccttggggcttgtggccgtcctgtgaggcattagttctccctctgagcctggaatctcttttgacgagtcatcatttttcacttttttacactgcatcttggctgcagcatgcctctgtcgttttcgcttccttggcttgtcaaatatcttggtagtgcctccaccaaaatcttttgaataagatgtggcacaagattcagttatgccattctccaggtgaccagcttcatagcactttttagaaaggccaaggtcccccttcttgggcataaatccagggtctaaatcattggattcaagaagtttcttagttggttttctttgacgtttactttcataatttcctggcgttttaactagcaattcctcagactcaagggcaggccgtggagagacttccggagccacaggcacagacaaggtcagctgcggcaactcagcatgtccacctccaagttctgactgagccaaggggccctccaaaaacggagcctccctttcaagaactggaggctcttctttggttgaaatcaaagaattctcgtccacctgcttgttctgagcactagatcgacctcgggctagaaggctttcctcttcacagcgggaacttaccttgtgcacctgctcctgtaccttcttttgttttttcttaggagcaaatatctgatcatattcttctgtatattccaaaagccacttgcttggcttcctaaggcgtttcttctctgaccgcacagctggttcagggagctcagcctgtggtgtcaaactgggaattcctggctccttttccatgtcaccaatgctggcactggatttatcacaaacatttaaccgtggcccagctgaatctaagcagtcagcatgattttgctctgtcagtggttcctcaagtatgcttgctgaaggagttctatgctctggaaactcatcccgcccctcctgcacagggtcactaggaagtaagaccctaaaggcacactcagagttttctttctctttaaatctgttcatgcgcttacgaggtttagtgcgcctttggtttaaacgctgccaccgctttttaggcaccacttgatttacaccattgagttcatcattctcactgttcattacagagtccagctctgggccttttccgttttcaaaagagagtcctttttcagaaattttaccaggatcagattgcttaaccttgctatcgaaatgcacatcagaaaaatggtcaccatcttcacttgttaagtggcccattatctgaaggggatcctctttactaggatcttctgccccacctctcaatgaacctccacgttctcggtctccctgcagtacagcatcaagagtcacacttggaagctgattcagttttcttttgcgctcggtctttaaggctttacggttcactgtgttctttaccatttgggctgaaaaagcatctcgcaatttggatgaaggctttgatcgtccacagttgcgcctagtaacacagtctgaacgacttttaccagaagcagggaggtctctcttgtcggacagtaagccaggtagggaagcagacaactcgccagataatgcagagtcacccccactagggctaggattggcggagttctgagtgccatctccctttttctctgaattgtgtgtggagcctcctgaaaccaaaaccttagagactcctacaggactattagtagaacagtccccacgaccaggactccggtaagagaccaggttttgagcagtcatcaaccgctgctccttcgtcttactatcatgcatatctttcaacatcattagcaatgtactgaatttgtagtctggttcaataggtatgtgattctgactagaagcagaagagaaaagtaatggttttgatggctttgatgttccagagtcactgacatcctcacctaaggatctgtaagagagttccttcaactcggataaaacatgtttcaccactgctgtttctatgtcacttgaatccctggttttctcatgcatattgttcagtagttttagaccatccactttcccacttttagaaatgctggccaaaggagagcctttggtatcagaagagcagcatttcaaactgcactcctcatttataactgggggttctgccataactggattttctttgtgtttgcactttatacttcggaacttgggctgtttgcttttcgaatgtaatagagcttgatttgctgccccaccctttattaacgagttctcactggatatgcttgatgacaggttgaattttggagagagagcatcatttgtaaaatctgactggggtttgtgaacaagagtagatgccttcagatcagagagattaacctgagacgtctcggttccaggctctgcactcttagtacaacccattaagtggtctgtatgtgagttactaatgagaggcttctgttttgcttttaccctagtgtttgtggcagcaaacctagaatactttatcttttcatttttctgcatagataacatgttctctgttctatcgaaagcatctggaatttcaaggacactgttatcagactctgagctgtgttctatgggatccaggtcactgcttccatcatcagaagtggtacagatactaatggaatcacttcgcttttcctcatcacctgctccaatatagcagagcttcacttttgaaccacacaccaggcttcgttggggtttattcttctctcgagaacactttgagatcaaagcaccctcaggcaagcccaataaagagtcaccatttgaagtctcaaattctttctttgcagtgttttttccacaggaagaaaacagaaaacttcctggggcagtgttggaccctgtgaggctatttgctatcctggaaagttcattagaggcctgcgtatcagatatatccccagagataaagtttaggccaaggttctctggaatctttcccctccgttcatctttatgtgcttcaaattgtatgtggccctttttcacactagtcctttttggattatcagagctctttctggctcgagatttagcgcaaggcttttccttctcatctgcagaatgttcagaatcaaaagccagtgatttcaaacagccattaagcaacaggtcatgttctgactcaggatcatttgtgcagtcttcaaatggcatatcttcttcactgtccaacttgattgaaccaggaatacattttcggttctttgaccccttgggaacatcatactgttctgcaagtccaacactggcttcccatttactcaaaattttctgaggaaccttatgcctatatcctttttctttctgtttccctcttctcctaaggacaggtagctcttcgaattgatgtctgccttcaaacatgacgattgcttttccagccacccaggctctctcagaaggatctccaaaagcctccacgtagtactgccgatagggcctccggttggaaactttcatttttgaatgtgtgttaatcaacggatcagaacaaatcctgcagggccaccatgggcgtctcttgaattttgcccagatgagatctccaacttcatacttcagtggcgtagactttttcttaggttgacaaaatggcaattcctgtgaagtagatgatgatgaagttccaggtaattctagcatgtttcctaatgtactggtactggaatctggatcatcctggagttcaggggagttattacaagagggttcctgtttcatagcaagtgctgtaggaccaccaggactcaaggaagtgcaaacaattggcgtctgagctcttgaatcacttttttcagggtcttgaaaggattctgatccatcagcagacccatttaaatactctacattgatcatggaggccaaatcctgtagtctccgcagtggaatgtaacaagatggagaatcttgtccataagcattttgggatgttccactgacagtcgataactgcatagtacacccattaagtggctcagaaaaattggattgaccattaccgaaagggctgtccttgtcttcaggggcatctaaattcactggattggaaaagggcagcagacaatttcttctgggtagttcacaggtctgatccatcctgggccggcatcaaccgtgccccgcgccccctcccgggccagctggggggagggggtgaccctcattacactggggtgcgagcggagcggtggggagagagcggggccgctcgccgcacccccctccccccgcgtctctcttcaggggagaaggcagcgagcgcgacctgccccggcctattccgccgccgcctcctcctcctcac

SEQ ID NO: 19174 - RNA, 11094 nt, Homo sapiens
  source 1..11094: mol_type = other RNA
tgtcttctctcctcccaaacaggaacccgggtttcttgagctgccagtccctcaacccttggcagtgcttatttataccgtgaaattagcaccatcattacattttattgtgtgtgtgtacaaaacaatgatctattcttatttcaatttacactatagcagcctctggccctgttgcactggccctaggaagctcagctgagaactaactggccatagccaatgacaggctcccacagcaactaccaagcagtgacttggaatgtctacacatggaactgctcaaatgaaactcagcaagaaaggggctggaggcagctccttctctgccatgatctgagagaggttaggacactgggctcctctaacctggctgataaaccccaagaggatgacagtatcatttaaaaaaccttagtaaaatccaccttatagggactaagggtaaaacctatccaagtttcatgctgtcctcattactccctatgggggaatctgtcaggactaaactttctgccattctgttctcatgaggcaacattagaattacaacctgggagtccggctccagtgagcagacagtgccgagcctgggaagggatcaacagggtgtttcatgccctgaccatagtgtggggtgaaggatgtaaagaataaaataactattttcatcaatgctaaagatttggttcagaagagggtcaacacagtgatttaagtcatctcaaactcagtaacagggtaaagcagacatttaaaaatgaggatgtttctgtatcaatgacagctattttgctattagactgggttggctccagcaagataagcaaatgaggctttgaatgtaaatttcaacatttttcataatctttttctgacttagcagggctagatgtattggctttctagctacccatggagaatttcaacttttgccttgtccctggaaaaggcctcctggggagctggctccaaggcaaacactcttgagatctcaatttccaagcacatacccaaataccaccctgcgttaaggaccagaagttttctaagatgaaagatttccttttcactccaattcacatccctttggaaaaggggtcttattacaaacttcaggggacgtcccacagggctggcaaggccactccctccccaccttcctccaagagtcacatttcccaacagttgttgtgactctgcttctaattggatagtgactgctttcatgattttaaccatctagtatcacatgctgctactggtgggcccaatagctcaaatttctagtttccagtggttttctagttcccattcaatggcccttgaaggaagcccagatgtccatccattcagatgaagaactgctccccaaaatggctcagaagctgttttcccaggcaggtctggaacgaagcctccaatgaatggcggagaatggaaagaaccaaaataaaaccacaaagcagccaatcatggcccctttccctcactccctcctgtcctgtgagacatctagactgctgtcaagttgattacctaccaaagcctactttagagaagctactttagaatcaaacttctccacggaaaatttttacatggcctgcacgccctccccccgccccccccaaattcacagtttatttcatgaaacaaagagctacggtaatttaacacacaacatagtgaaaggagactctgacagtgcagtgcagatacctttttctgatcacaactacagatgactggagagaaaagggcacaggactggcaccaagcaaaccctactcatatgacctaaaagattagggaaagggacctactagctgcagttatatatttattattctcacacatgataaatacttaatataatgaactttaatgttctcggtgaatttctttaaaaatatctttttcatggtttaaaattcttttaaaagaaaataagatgctttacgttttctcttccttttgaacaaagagcttttcctctttgatgatgtgggaagagagagaggatgaaaggggagaactaggcaggtggaattcacagaggagattccgaggtctcagtgaaatgcagggataggcccctaaactcaggacagccctgcccagcctcgtccctctgcctgagttcaagtgtctcaacctcagagacagactttgggaaataaaagcagattctatttttaatctttagataaagcgcaaatgcttctataataactactgttccctccgtggaattgatgggagtaacctcaataagaacttgaggaaattgggaccaaatacagaatcctattgagagcgtgaaagccataactaagagataatggccaggagacgttagggccggggatggcctgctggctaagttggcaaagcagagaggtaaacatgttggtctaaggacaaaggaggggtagacaagtgggaggaaactagccaaacagcacttcctgttggcagtctgtgagctgggtgaatggtagggcagggtagcaccaacagatttcccagcccttgggccccagctcagggcagcagtaacagataatcagcagttaataggagtcatctcttagcctggacgttgctctaaacaccacctcttgccagtcttcagggaagggttctggcttgcctttgagctaagtcagcaggcaggtgctctcaatacagagcacagcaattctcagggaggcgaagaagaggactccctccactcaggagggaaaaggaatggggaaaagaaatttcccatcaggatctggtactcttcctgaagctggtgtgtctagctcagagcttgccagagattccctatgtccactgcccgaggctctgaaatctgaaagcacctgagtgttttagggaaatagggatggggtggattcatgtacaaagagaaaaataggtagaaacaaaagcaaagaaagagaagcttgccaaatgccttcttccactgctggaaatctacattcgcacagagcccgactgcccctgaccacctgctcctccaaggactgatcttgagactctgcacagcccagacaaaagcagcagcggcgaccccacagccaacagccttgctggcctcaatgcagcacccttgcatctatagaggagacctctgtgagtgtgcgcgcatgcacacgcacccatgcacaccgcagccaagagacacttcctcaacacaaccacttctggtgccacaaaggacatttcaaaatgagtctaaagccccagggcccctcagaacttcctgttacttcctggtcaaaggttcctgaaagccttggaatccaggctcacagggatgaggcctgtatctctcatcagtgactagcacccggcctagaacacgtgaatgctcaggaaatcgccactgatttgaaagaacaccatttcctcccaagggttcctaggtgccctcaatggggctctgtctggttggggaaatcgctttgagagcccctataccttccaacctgaccagcggaattgaattccatacttgactccagagtggactttttatttcacgatgaccatgtggaaaagttgggggaaagagacccaagtctgtctgtctccttggttggggcccactggattttcatacatggttcacacaaccataagcccccactggctaatgtcacaagagttctgagtgttgggatatgaggaaagaataacagtgggaaagtgttcggggcagatgtgtttttttttaagggggaaagaaagaaaagatttcccctccccaaatggtaccctgggggcagcttgtttgttcatgtgacattgattggtactacttctgttctgattctgcacacttgtgactggaaggagcctggttaagagctggaagtgtattttgctctggtttggggtcttgccctcttccaagagaccagcaagtctgtgccaatgtctgtgtgctcccagcagaccagcaagactgtgccagtgtctgtccagccactatgggccagagccctgcccgtgatgaggcttttcccagggcccagggactttgctctgtggttaccaacttcttttcttcagtggggagggaggctggggccttcccgagagacctaaaagattgcccactcttggcggcaagtgcaggtagttgctggcctccgaccatctgcttcgcctgcttcaccaggcccggggattggctaagaggccctggggtctgctcagcccctgcagaagctcttcctgaggcctgagttgttggctcatataaaaaggccttggcaggaggctgagaaagaagtctggcctgggtgagtgatttaacagcttgccaggggtcctctgaaggggctgctgctttcccagatgtctgaagaggatctgacacacagcctttctcaacagctctcggcatatgccccagacctttgctggcaggccatgaacttgactccaacactggcatcttctcatcagcctgtggtgtgacctgatgaggtgaagctgcccgctccttctggcgaggagttaggtctatgagatccatcaccaaagcagctctattttttgactgagtattctggtccacaggcctcagtgctttttctttagctacaagggtctggaccacagctgatagtactttctcaggaggtgggagtctctgggacaaagaggcatggggtttgtcagtaggcctgtctgaagtctggggtttgggactgctagtaatgagcagtctgtctggcggcggaagtctcaggccagtgggaactgaggttttctccagtgactggggccttgggctggcagcacctatggatttatccagccttgggtcagccgtccccagaggtctttccagtggttgggacctgactgagggtgaggagcttgggctggtcactggagagggtttgtcgcttagctggggtcttggtcctgccactgctggtggcctgtccagtggcctctggctggaaaccaaggattgggatttggtccctgacccagcgaggtctctgaccttatctaaaggctggggcctggagtcagttctctcaagaggtctttcaggtagcaatggcctctgacaagtccctgccagagcttttttggagagcgacagcatctggttggtgtcagcaggaggtttatctgacattttgggtgcctgagcagccattcctgttgattgctctgccaggtgagtgcttggccctggaggcagcggtactgggggaggcacatactcacggatctccccaggttccagaggattgggcccacaggggtcatgctcagtacaagacagacgcccatccagtttggaaatgaaaagcatcccttctcgatgctgcttacaaaaggagctggggcacatctcacagaaggaggctgcttccttcccgcagatgtcacactgatgccacggacattcccatttccctgctggtcgcttggtcagattgagacagtctgcgtggtaaacttttgggcagcctggtttcttgcaggagacgagctggccagcatccccacaactaaaacactcatcttctcgctcctttgtgatttcaccctgggtcctgcgctttccctgttgcttcttcttgaatttctttgacttttcttccgtggcaatgggttgattctttggccttacacccaagaagccactgcagttcggggctccacatttgcaaacagtctttccattcccaagacattctaggttgtagttgaaggtaagttcagtgcctgctttaatgtcacttagtgcaaaaaggcctacacgggtatctccattcacagaccacttctgtgtttcacagttgggctggcagcaatgattcatgaaccgagcatagtttcctttgggaccagcatcaatgattcggtctttgtctagggtgagcatatagaaattagtgatatcatgttcttgagcatagcgaattcgagctctgcattcttcttcatctataagctcacccacatactcattcacaaattcaccctttttaatatctgtttttgtccgtagaccccaaccccgctgtaatgtgcggaaaatttcaacctctggatattggcgcttggaaaagcactggttttgacagcgccctccggcaggacacactgtggggtggcactcatagagcagcatgcggttgatgcattcagagtctatcccacaggggttctcatcagtagctttacagttgcaacggggtatttcagataagtctgcagtgaagatctgtaccctgccaataggacggtttacctttatatgtttataaggtggtggcttcttgtcattctttcggtcttcctgcagctgtcttagctctttttgggcctttaattcctcaaaccttgctgcagcttcctgaagagcttttttatatgtcccatccactcctttgcccatcttatccttgctgctcacgtcaccctccatgtaagggaagactcgggcctggtgagtccacaaatagtcattagatccaaaaaagaggactgggaactctcccacatcatgtctcatcttatcaatgttggaaggaacagctcgaggatggcagatctcagctggccaccacctgtatcgtccaacttttacccagacaatctccctgtagtgtggctttttgcctgctttacagtcattgcaataccagtttccttcagggatatcaatgttcaggcattcacgatgaaaagcagcagggcaagaatcacagcacagaaggctgcctccttctgagcacacaaagcaccagctaacattaacatgctcatgatttcggcagccccgcctaggggtaaagtgattagggcagatgatactattagatgcaaggatctttgacccagcagccaggcaaaagtcattggcgtggtatgccacaggacagcggacacagcgcatcaaccgacctttagatgcagaaacattggctggattagcagcatgacaggttatacagatgtggagggagcaccggaagcccttgttctgcataacagtgggtgggtacttctggacacactcttcatggtaaaactttccacacaagggtagaaggcaccttttaacatcttccccactctgcttacatacaaaacaggtatggattcctgtgcgacattcattgcagataaattttcctcttggcatctcagtcaatccaaggcactccaggtggaaagccccacagcactgagcctcacataacagcagctcacccaatttttcacaattctgacagacattctccttgagtgcagctcctccaccgcgttcaccctgcatttttttagaggcaggcatcccgggatcgtgttctacaccttcctcaacagtctccttggggcttgtggccgtcctgtgaggcattagttctccctctgagcctggaatctcttttgacgagtcatcatttttcacttttttacactgcatcttggctgcagcatgcctctgtcgttttcgcttccttggcttgtcaaatatcttggtagtgcctccaccaaaatcttttgaataagatgtggcacaagattcagttatgccattctccaggtgaccagcttcatagcactttttagaaaggccaaggtcccccttcttgggcataaatccagggtctaaatcattggattcaagaagtttcttagttggttttctttgacgtttactttcataatttcctggcgttttaactagcaattcctcagactcaagggcaggccgtggagagacttccggagccacaggcacagacaaggtcagctgcggcaactcagcatgtccacctccaagttctgactgagccaaggggccctccaaaaacggagcctccctttcaagaactggaggctcttctttggttgaaatcaaagaattctcgtccacctgcttgttctgagcactagatcgacctcgggctagaaggctttcctcttcacagcgggaacttaccttgtgcacctgctcctgtaccttcttttgttttttcttaggagcaaatatctgatcatattcttctgtatattccaaaagccacttgcttggcttcctaaggcgtttcttctctgaccgcacagctggttcagggagctcagcctgtggtgtcaaactgggaattcctggctccttttccatgtcaccaatgctggcactggatttatcacaaacatttaaccgtggcccagctgaatctaagcagtcagcatgattttgctctgtcagtggttcctcaagtatgcttgctgaaggagttctatgctctggaaactcatcccgcccctcctgcacagggtcactaggaagtaagaccctaaaggcacactcagagttttctttctctttaaatctgttcatgcgcttacgaggtttagtgcgcctttggtttaaacgctgccaccgctttttaggcaccacttgatttacaccattgagttcatcattctcactgttcattacagagtccagctctgggccttttccgttttcaaaagagagtcctttttcagaaattttaccaggatcagattgcttaaccttgctatcgaaatgcacatcagaaaaatggtcaccatcttcacttgttaagtggcccattatctgaaggggatcctctttactaggatcttctgccccacctctcaatgaacctccacgttctcggtctccctgcagtacagcatcaagagtcacacttggaagctgattcagttttcttttgcgctcggtctttaaggctttacggttcactgtgttctttaccatttgggctgaaaaagcatctcgcaatttggatgaaggctttgatcgtccacagttgcgcctagtaacacagtctgaacgacttttaccagaagcagggaggtctctcttgtcggacagtaagccaggtagggaagcagacaactcgccagataatgcagagtcacccccactagggctaggattggcggagttctgagtgccatctccctttttctctgaattgtgtgtggagcctcctgaaaccaaaaccttagagactcctacaggactattagtagaacagtccccacgaccaggactccggtaagagaccaggttttgagcagtcatcaaccgctgctccttcgtcttactatcatgcatatctttcaacatcattagcaatgtactgaatttgtagtctggttcaataggtatgtgattctgactagaagcagaagagaaaagtaatggttttgatggctttgatgttccagagtcactgacatcctcacctaaggatctgtaagagagttccttcaactcggataaaacatgtttcaccactgctgtttctatgtcacttgaatccctggttttctcatgcatattgttcagtagttttagaccatccactttcccacttttagaaatgctggccaaaggagagcctttggtatcagaagagcagcatttcaaactgcactcctcatttataactgggggttctgccataactggattttctttgtgtttgcactttatacttcggaacttgggctgtttgcttttcgaatgtaatagagcttgatttgctgccccaccctttattaacgagttctcactggatatgcttgatgacaggttgaattttggagagagagcatcatttgtaaaatctgactggggtttgtgaacaagagtagatgccttcagatcagagagattaacctgagacgtctcggttccaggctctgcactcttagtacaacccattaagtggtctgtatgtgagttactaatgagaggcttctgttttgcttttaccctagtgtttgtggcagcaaacctagaatactttatcttttcatttttctgcatagataacatgttctctgttctatcgaaagcatctggaatttcaaggacactgttatcagactctgagctgtgttctatgggatccaggtcactgcttccatcatcagaagtggtacagatactaatggaatcacttcgcttttcctcatcacctgctccaatatagcagagcttcacttttgaaccacacaccaggcttcgttggggtttattcttctctcgagaacactttgagatcaaagcaccctcaggcaagcccaataaagagtcaccatttgaagtctcaaattctttctttgcagtgttttttccacaggaagaaaacagaaaacttcctggggcagtgttggaccctgtgaggctatttgctatcctggaaagttcattagaggcctgcgtatcagatatatccccagagataaagtttaggccaaggttctctggaatctttcccctccgttcatctttatgtgcttcaaattgtatgtggccctttttcacactagtcctttttggattatcagagctctttctggctcgagatttagcgcaaggcttttccttctcatctgcagaatgttcagaatcaaaagccagtgatttcaaacagccattaagcaacaggtcatgttctgactcaggatcatttgtgcagtcttcaaatggcatatcttcttcactgtccaacttgattgaaccaggaatacattttcggttctttgaccccttgggaacatcatactgttctgcaagtccaacactggcttcccatttactcaaaattttctgaggaaccttatgcctatatcctttttctttctgtttccctcttctcctaaggacaggtagctcttcgaattgatgtctgccttcaaacatgacgattgcttttccagccacccaggctctctcagaaggatctccaaaagcctccacgtagtactgccgatagggcctccggttggaaactttcatttttgaatgtgtgttaatcaacggatcagaacaaatcctgcagggccaccatgggcgtctcttgaattttgcccagatgagatctccaacttcatacttcagtggcgtagactttttcttaggttgacaccctcacaaccttacaagacagcattatctcgattttgcagataaagaaactgaggctcaaaaaggttaagtcacaggctgggtgcggtggctcatgc

SEQ ID NO: 19175 - RNA, 10771 nt, Homo sapiens
  source 1..10771: mol_type = other RNA
tgtcttctctcctcccaaacaggaacccgggtttcttgagctgccagtccctcaacccttggcagtgcttatttataccgtgaaattagcaccatcattacattttattgtgtgtgtgtacaaaacaatgatctattcttatttcaatttacactatagcagcctctggccctgttgcactggccctaggaagctcagctgagaactaactggccatagccaatgacaggctcccacagcaactaccaagcagtgacttggaatgtctacacatggaactgctcaaatgaaactcagcaagaaaggggctggaggcagctccttctctgccatgatctgagagaggttaggacactgggctcctctaacctggctgataaaccccaagaggatgacagtatcatttaaaaaaccttagtaaaatccaccttatagggactaagggtaaaacctatccaagtttcatgctgtcctcattactccctatgggggaatctgtcaggactaaactttctgccattctgttctcatgaggcaacattagaattacaacctgggagtccggctccagtgagcagacagtgccgagcctgggaagggatcaacagggtgtttcatgccctgaccatagtgtggggtgaaggatgtaaagaataaaataactattttcatcaatgctaaagatttggttcagaagagggtcaacacagtgatttaagtcatctcaaactcagtaacagggtaaagcagacatttaaaaatgaggatgtttctgtatcaatgacagctattttgctattagactgggttggctccagcaagataagcaaatgaggctttgaatgtaaatttcaacatttttcataatctttttctgacttagcagggctagatgtattggctttctagctacccatggagaatttcaacttttgccttgtccctggaaaaggcctcctggggagctggctccaaggcaaacactcttgagatctcaatttccaagcacatacccaaataccaccctgcgttaaggaccagaagttttctaagatgaaagatttccttttcactccaattcacatccctttggaaaaggggtcttattacaaacttcaggggacgtcccacagggctggcaaggccactccctccccaccttcctccaagagtcacatttcccaacagttgttgtgactctgcttctaattggatagtgactgctttcatgattttaaccatctagtatcacatgctgctactggtgggcccaatagctcaaatttctagtttccagtggttttctagttcccattcaatggcccttgaaggaagcccagatgtccatccattcagatgaagaactgctccccaaaatggctcagaagctgttttcccaggcaggtctggaacgaagcctccaatgaatggcggagaatggaaagaaccaaaataaaaccacaaagcagccaatcatggcccctttccctcactccctcctgtcctgtgagacatctagactgctgtcaagttgattacctaccaaagcctactttagagaagctactttagaatcaaacttctccacggaaaatttttacatggcctgcacgccctccccccgccccccccaaattcacagtttatttcatgaaacaaagagctacggtaatttaacacacaacatagtgaaaggagactctgacagtgcagtgcagatacctttttctgatcacaactacagatgactggagagaaaagggcacaggactggcaccaagcaaaccctactcatatgacctaaaagattagggaaagggacctactagctgcagttatatatttattattctcacacatgataaatacttaatataatgaactttaatgttctcggtgaatttctttaaaaatatctttttcatggtttaaaattcttttaaaagaaaataagatgctttacgttttctcttccttttgaacaaagagcttttcctctttgatgatgtgggaagagagagaggatgaaaggggagaactaggcaggtggaattcacagaggagattccgaggtctcagtgaaatgcagggataggcccctaaactcaggacagccctgcccagcctcgtccctctgcctgagttcaagtgtctcaacctcagagacagactttgggaaataaaagcagattctatttttaatctttagataaagcgcaaatgcttctataataactactgttccctccgtggaattgatgggagtaacctcaataagaacttgaggaaattgggaccaaatacagaatcctattgagagcgtgaaagccataactaagagataatggccaggagacgttagggccggggatggcctgctggctaagttggcaaagcagagaggtaaacatgttggtctaaggacaaaggaggggtagacaagtgggaggaaactagccaaacagcacttcctgttggcagtctgtgagctgggtgaatggtagggcagggtagcaccaacagatttcccagcccttgggccccagctcagggcagcagtaacagataatcagcagttaataggagtcatctcttagcctggacgttgctctaaacaccacctcttgccagtcttcagggaagggttctggcttgcctttgagctaagtcagcaggcaggtgctctcaatacagagcacagcaattctcagggaggcgaagaagaggactccctccactcaggagggaaaaggaatggggaaaagaaatttcccatcaggatctggtactcttcctgaagctggtgtgtctagctcagagcttgccagagattccctatgtccactgcccgaggctctgaaatctgaaagcacctgagtgttttagggaaatagggatggggtggattcatgtacaaagagaaaaataggtagaaacaaaagcaaagaaagagaagcttgccaaatgccttcttccactgctggaaatctacattcgcacagagcccgactgcccctgaccacctgctcctccaaggactgatcttgagactctgcacagcccagacaaaagcagcagcggcgaccccacagccaacagccttgctggcctcaatgcagcacccttgcatctatagaggagacctctgtgagtgtgcgcgcatgcacacgcacccatgcacaccgcagccaagagacacttcctcaacacaaccacttctggtgccacaaaggacatttcaaaatgagtctaaagccccagggcccctcagaacttcctgttacttcctggtcaaaggttcctgaaagccttggaatccaggctcacagggatgaggcctgtatctctcatcagtgactagcacccggcctagaacacgtgaatgctcaggaaatcgccactgatttgaaagaacaccatttcctcccaagggttcctaggtgccctcaatggggctctgtctggttggggaaatcgctttgagagcccctataccttccaacctgaccagcggaattgaattccatacttgactccagagtggactttttatttcacgatgaccatgtggaaaagttgggggaaagagacccaagtctgtctgtctccttggttggggcccactggattttcatacatggttcacacaaccataagcccccactggctaatgtcacaagagttctgagtgttgggatatgaggaaagaataacagtgggaaagtgttcggggcagatgtgtttttttttaagggggaaagaaagaaaagatttcccctccccaaatggtaccctgggggcagcttgtttgttcatgtgacattgattggtactacttctgttctgattctgcacacttgtgactggaaggagcctggttaagagctggaagtgtattttgctctggtttggggtcttgccctcttccaagagaccagcaagtctgtgccaatgtctgtgtgctcccagcagaccagcaagactgtgccagtgtctgtccagccactatgggccagagccctgcccgtgatgaggcttttcccagggcccagggactttgctctgtggttaccaacttcttttcttcagtggggagggaggctggggccttcccgagagacctaaaagattgcccactcttggcggcaagtgcaggtagttgctggcctccgaccatctgcttcgcctgcttcaccaggcccggggattggctaagaggccctggggtctgctcagcccctgcagaagctcttcctgaggcctgagttgttggctcatataaaaaggccttggcaggaggctgagaaagaagtctggcctgggtgagtgatttaacagcttgccaggggtcctctgaaggggctgctgctttcccagatgtctgaagaggatctgacacacagcctttctcaacagctctcggcatatgccccagacctttgctggcaggccatgaacttgactccaacactggcatcttctcatcagcctgtggtgtgacctgatgaggtgaagctgcccgctccttctggcgaggagttaggtctatgagatccatcaccaaagcagctctattttttgactgagtattctggtccacaggcctcagtgctttttctttagctacaagggtctggaccacagctgatagtactttctcaggaggtgggagtctctgggacaaagaggcatggggtttgtcagtaggcctgtctgaagtctggggtttgggactgctagtaatgagcagtctgtctggcggcggaagtctcaggccagtgggaactgaggttttctccagtgactggggccttgggctggcagcacctatggatttatccagccttgggtcagccgtccccagaggtctttccagtggttgggacctgactgagggtgaggagcttgggctggtcactggagagggtttgtcgcttagctggggtcttggtcctgccactgctggtggcctgtccagtggcctctggctggaaaccaaggattgggatttggtccctgacccagcgaggtctctgaccttatctaaaggctggggcctggagtcagttctctcaagaggtctttcaggtagcaatggcctctgacaagtccctgccagagcttttttggagagcgacagcatctggttggtgtcagcaggaggtttatctgacattttgggtgcctgagcagccattcctgttgattgctctgccaggtgagtgcttggccctggaggcagcggtactgggggaggcacatactcacggatctccccaggttccagaggattgggcccacaggggtcatgctcagtacaagacagacgcccatccagtttggaaatgaaaagcatcccttctcgatgctgcttacaaaaggagctggggcacatctcacagaaggaggctgcttccttcccgcagatgtcacactgatgccacggacattcccatttccctgctggtcgcttggtcagattgagacagtctgcgtggtaaacttttgggcagcctggtttcttgcaggagacgagctggccagcatccccacaactaaaacactcatcttctcgctcctttgtgatttcaccctgggtcctgcgctttccctgttgcttcttcttgaatttctttgacttttcttccgtggcaatgggttgattctttggccttacacccaagaagccactgcagttcggggctccacatttgcaaacagtctttccattcccaagacattctaggttgtagttgaaggtaagttcagtgcctgctttaatgtcacttagtgcaaaaaggcctacacgggtatctccattcacagaccacttctgtgtttcacagttgggctggcagcaatgattcatgaaccgagcatagtttcctttgggaccagcatcaatgattcggtctttgtctagggtgagcatatagaaattagtgatatcatgttcttgagcatagcgaattcgagctctgcattcttcttcatctataagctcacccacatactcattcacaaattcaccctttttaatatctgtttttgtccgtagaccccaaccccgctgtaatgtgcggaaaatttcaacctctggatattggcgcttggaaaagcactggttttgacagcgccctccggcaggacacactgtggggtggcactcatagagcagcatgcggttgatgcattcagagtctatcccacaggggttctcatcagtagctttacagttgcaacggggtatttcagataagtctgcagtgaagatctgtaccctgccaataggacggtttacctttatatgtttataaggtggtggcttcttgtcattctttcggtcttcctgcagctgtcttagctctttttgggcctttaattcctcaaaccttgctgcagcttcctgaagagcttttttatatgtcccatccactcctttgcccatcttatccttgctgctcacgtcaccctccatgtaagggaagactcgggcctggtgagtccacaaatagtcattagatccaaaaaagaggactgggaactctcccacatcatgtctcatcttatcaatgttggaaggaacagctcgaggatggcagatctcagctggccaccacctgtatcgtccaacttttacccagacaatctccctgtagtgtggctttttgcctgctttacagtcattgcaataccagtttccttcagggatatcaatgttcaggcattcacgatgaaaagcagcagggcaagaatcacagcacagaaggctgcctccttctgagcacacaaagcaccagctaacattaacatgctcatgatttcggcagccccgcctaggggtaaagtgattagggcagatgatactattagatgcaaggatctttgacccagcagccaggcaaaagtcattggcgtggtatgccacaggacagcggacacagcgcatcaaccgacctttagatgcagaaacattggctggattagcagcatgacaggttatacagatgtggagggagcaccggaagcccttgttctgcataacagtgggtgggtacttctggacacactcttcatggtaaaactttccacacaagggtagaaggcaccttttaacatcttccccactctgcttacatacaaaacaggtatggattcctgtgcgacattcattgcagataaattttcctcttggcatctcagtcaatccaaggcactccaggtggaaagccccacagcactgagcctcacataacagcagctcacccaatttttcacaattctgacagacattctccttgagtgcagctcctccaccgcgttcaccctgcatttttttagaggcaggcatcccgggatcgtgttctacaccttcctcaacagtctccttggggcttgtggccgtcctgtgaggcattagttctccctctgagcctggaatctcttttgacgagtcatcatttttcacttttttacactgcatcttggctgcagcatgcctctgtcgttttcgcttccttggcttgtcaaatatcttggtagtgcctccaccaaaatcttttgaataagatgtggcacaagattcagttatgccattctccaggtgaccagcttcatagcactttttagaaaggccaaggtcccccttcttgggcataaatccagggtctaaatcattggattcaagaagtttcttagttggttttctttgacgtttactttcataatttccttgtgcacctgctcctgtaccttcttttgttttttcttaggagcaaatatctgatcatattcttctgtatattccaaaagccacttgcttggcttcctaaggcgtttcttctctgaccgcacagctggttcagggagctcagcctgtggtgtcaaactgggaattcctggctccttttccatgtcaccaatgctggcactggatttatcacaaacatttaaccgtggcccagctgaatctaagcagtcagcatgattttgctctgtcagtggttcctcaagtatgcttgctgaaggagttctatgctctggaaactcatcccgcccctcctgcacagggtcactaggaagtaagaccctaaaggcacactcagagttttctttctctttaaatctgttcatgcgcttacgaggtttagtgcgcctttggtttaaacgctgccaccgctttttaggcaccacttgatttacaccattgagttcatcattctcactgttcattacagagtccagctctgggccttttccgttttcaaaagagagtcctttttcagaaattttaccaggatcagattgcttaaccttgctatcgaaatgcacatcagaaaaatggtcaccatcttcacttgttaagtggcccattatctgaaggggatcctctttactaggatcttctgccccacctctcaatgaacctccacgttctcggtctccctgcagtacagcatcaagagtcacacttggaagctgattcagttttcttttgcgctcggtctttaaggctttacggttcactgtgttctttaccatttgggctgaaaaagcatctcgcaatttggatgaaggctttgatcgtccacagttgcgcctagtaacacagtctgaacgacttttaccagaagcagggaggtctctcttgtcggacagtaagccaggtagggaagcagacaactcgccagataatgcagagtcacccccactagggctaggattggcggagttctgagtgccatctccctttttctctgaattgtgtgtggagcctcctgaaaccaaaaccttagagactcctacaggactattagtagaacagtccccacgaccaggactccggtaagagaccaggttttgagcagtcatcaaccgctgctccttcgtcttactatcatgcatatctttcaacatcattagcaatgtactgaatttgtagtctggttcaataggtatgtgattctgactagaagcagaagagaaaagtaatggttttgatggctttgatgttccagagtcactgacatcctcacctaaggatctgtaagagagttccttcaactcggataaaacatgtttcaccactgctgtttctatgtcacttgaatccctggttttctcatgcatattgttcagtagttttagaccatccactttcccacttttagaaatgctggccaaaggagagcctttggtatcagaagagcagcatttcaaactgcactcctcatttataactgggggttctgccataactggattttctttgtgtttgcactttatacttcggaacttgggctgtttgcttttcgaatgtaatagagcttgatttgctgccccaccctttattaacgagttctcactggatatgcttgatgacaggttgaattttggagagagagcatcatttgtaaaatctgactggggtttgtgaacaagagtagatgccttcagatcagagagattaacctgagacgtctcggttccaggctctgcactcttagtacaacccattaagtggtctgtatgtgagttactaatgagaggcttctgttttgcttttaccctagtgtttgtggcagcaaacctagaatactttatcttttcatttttctgcatagataacatgttctctgttctatcgaaagcatctggaatttcaaggacactgttatcagactctgagctgtgttctatgggatccaggtcactgcttccatcatcagaagtggtacagatactaatggaatcacttcgcttttcctcatcacctgctccaatatagcagagcttcacttttgaaccacacaccaggcttcgttggggtttattcttctctcgagaacactttgagatcaaagcaccctcaggcaagcccaataaagagtcaccatttgaagtctcaaattctttctttgcagtgttttttccacaggaagaaaacagaaaacttcctggggcagtgttggaccctgtgaggctatttgctatcctggaaagttcattagaggcctgcgtatcagatatatccccagagataaagtttaggccaaggttctctggaatctttcccctccgttcatctttatgtgcttcaaattgtatgtggccctttttcacactagtcctttttggattatcagagctctttctggctcgagatttagcgcaaggcttttccttctcatctgcagaatgttcagaatcaaaagccagtgatttcaaacagccattaagcaacaggtcatgttctgactcaggatcatttgtgcagtcttcaaatggcatatcttcttcactgtccaacttgattgaaccaggaatacattttcggttctttgaccccttgggaacatcatactgttctgcaagtccaacactggcttcccatttactcaaaattttctgaggaaccttatgcctatatcctttttctttctgtttccctcttctcctaaggacaggtagctcttcgaattgatgtctgccttcaaacatgacgattgcttttccagccacccaggctctctcagaaggatctccaaaagcctccacgtagtactgccgatagggcctccggttggaaactttcatttttgaatgtgtgttaatcaacggatcagaacaaatcctgcagggccaccatgggcgtctcttgaattttgcccagatgagatctccaacttcatacttcagtggcgtagactttttcttaggttgacaaaatggcaattcctgtgaagtagatgatgatgaagttccaggtaat

SEQ ID NO: 19176 - RNA, 2152 nt, Homo sapiens
  source 1..2152: mol_type = other RNA
tgtcttctctcctcccaaacaggattcaagtttccaaaaatggtcttggtacgcttcttagttttgctgacttgcacagtcacgtaagggtcactggatcctgttttgtccttggcttgtaggccctgggcacacaccacagtaatggtgatcttggctgaccatttggaggtgccatccagtacactctgcttcactgttttcatctgctgcacatgggcagctttgttcactgtgaagacgtcccggataacttcaaagatctctggcttatttcgctctcggatcttcatgcggtccttcatggccatgataatgttctgggtccggtcctcagctccatgtttacagctcttttctgcagcccgctgcaggcagtcagcattgagcagatcctggcacttctcatggcacttgactccacattcgctgcagcgcatgccctgccgggcaatgccccagagcaggccttcacactcatagcagtaggttggggtagtggccgtccagacctcaaagttatgaggagtggtgcacgaaatggggtagattaaggcctgcagggttttcttatacacgtgggatttcagctcttcgtccttaagagaagtgcgtgtagccattgcagaagtgattcctgccttccgagactggaccagtgacagatcactgacaagtggcagtggcttctttctgcgtaaatctggcatgctgtcaatgccatagagccctccggctggcccttccgggagccactgaggcagagaggggtcaccatcatctggaatctcctgcagctggagtcgaaccttggtaactgctcggatccaatgtgctctggcttgggtaaatggtgaagatgcattctcctcaggaaaactctcctggggacctaggaagtggtctttttgcagcaccagatctgggggagggtgggttgtggcatcttctttcatctccttgggttcacatgctgcctccttctctgcttgacctgtcacctccaagggtttctcttgttctccaaaacctgcttggccatctctggacaggctgtgagagctgtggcaagaatgaatcgagtccgtctcccgatggtcgtcatcttgttcgtgatactggtctagttcacttagctgagagcttccttgactcacattacaggaggagccatacctactgctgctggtggggctgatagcccgccgctctggataatcaaggtcataactttgcatagagtcattacaagagtcccgggaactgccttgaagtagcagctgctgtggcgatcgcaccggcacagggaactggtgcacagaagcgttgggctgggaagctgtatggtaaggaggtgggaagctgttgctggtctcactgcgatagtcactatctcggtcatcgacggcactatcagggtcttcaaaagaacactgggcggcagcagtgggcaatggcttcctctggctttcttcttgactagaatactcattgtcagctcccaaggcattgatttgctcccatttgtaggtccaatatctggcttcctcctctgggatatcaaaaggcaactcaaatcttgtatcaagcaaaattttatgaggagttgggtttctagttccacagatctcatcgtctttcattaacgtctctgcctctaatgtggaccattccccaggcccttcctcatccgactgacgaatagtcttcagcgcaatccacacagtccccaccatggtgtcccagatcagtcctttgttccatacctccacacttagacccaggtccaggcgactaatctcaaacatgaaatcctgttcccaggaaggctgatcaccacgaactgctacagttgtgctcttcacattctgtactttcagggtcacatatgtgttaaatttatctggtgaaccctggaatttggcccttttaacaatgttagaactaggtttagattgttaaatctaaacctggagaaaaaaagctgagacttctgatcaaaacttgaaaggcaaagagtcagacgagaccttaaaagtcaatctgatctcatatccaatgcaaaaatctctgttccaggctcctgacaacaaggtggagagatctaagttactcctgtggcaggcagccagtttcatgtgagatatcttct

SEQ ID NO: 19177 - RNA, 2230 nt, Homo sapiens
  source 1..2230: mol_type = other RNA
tgtcttctctcctcccaaacaggattcaagtttccaaaaatggtcttggtacgcttcttagttttgctgacttgcacagtcacgtaagggtcactggatcctgttttgtccttggcttgtaggccctgggcacacaccacagtaatggtgatcttggctgaccatttggaggtgccatccagtacactctgcttcactgttttcatctgctgcacatgggcagctttgttcactgtgaagacgtcccggataacttcaaagatctctggcttatttcgctctcggatcttcatgcggtccttcatggccatgataatgttctgggtccggtcctcagctccatgtttacagctcttttctgcagcccgctgcaggcagtcagcattgagcagatcctggcacttctcatggcacttgactccacattcgctgcagcgcatgccctgccgggcaatgccccagagcaggccttcacactcatagcagtaggttggggtagtggccgtccagacctcaaagttatgaggagtggtgcacgaaatggggtagattaaggcctgcagggttttcttatacacgtgggatttcagctcttcgtccttaagagaagtgcgtgtagccattgcagaagtgattcctgccttccgagactggaccagtgacagatcactgacaagtggcagtggcttctttctgcgtaaatctggcatgctgtcaatgccatagagccctccggctggcccttccgggagccactgaggcagagaggggtcaccatcatctggaatctcctgcagctggagtcgaaccttggtaactgctcggatccaatgtgctctggcttgggtaaatggtgaagatgcattctcctcaggaaaactctcctggggacctaggaagtggtctttttgcagcaccagatctgggggagggtgggttgtggcatcttctttcatctccttgggttcacatgctgcctccttctctgcttgacctgtcacctccaagggtttctcttgttctccaaaacctgcttggccatctctggacaggctgtgagagctgtggcaagaatgaatcgagtccgtctcccgatggtcgtcatcttgttcgtgatactggtctagttcacttagctgagagcttccttgactcacattacaggaggagccatacctactgctgctggtggggctgatagcccgccgctctggataatcaaggtcataactttgcatagagtcattacaagagtcccgggaactgccttgaagtagcagctgctgtggcgatcgcaccggcacagggaactggtgcacagaagcgttgggctgggaagctgtatggtaaggaggtgggaagctgttgctggtctcactgcgatagtcactatctcggtcatcgacggcactatcagggtcttcaaaagaacactgggcggcagcagtgggcaatggcttcctctggctttcttcttgactagaatactcattgtcagctcccaaggcattgatttgctcccatttgtaggtccaatatctggcttcctcctctgggatatcaaaaggcaactcaaatcttgtatcaagcaaaattttatgaggagttgggtttctagttccacagatctcatcgtctttcattaacgtctctgcctctaatgtggaccattccccaggcccttcctcatccgactgacgaatagtcttcagcgcaatccacacagtccccaccatggtgtcccagatcagtcctttgttccatacctccacacttagacccaggtccaggcgactaatctcaaacatgaaatcctgttcccaggaaggctgatcaccacgaactgctacagttgtgctcttcacattctgtactttcagggtcacatatgtgttaaatttatctggtgaaccctggaatttggcccttttaacgcgcacgcagagcagtgacatggccgaggatcgggcaagcctctgccgcgccccagccgcgccggaccgctccctctttcctctcagcaggtgccgcgactgctctcgttaccggccccacgggtctggcagctcctcatggtcccggtcgcaggtagcgtcccgccgctgcctcggacccgccccaaatctcaccgtctgagcgaactccgggtagcggtgagtaccggccggcaggctggggactgggcgcggcacagcgacgccatcgctgggaggtaggagctgccgggact

SEQ ID NO: 19178 - RNA, 2266 nt, Homo sapiens
  source 1..2266: mol_type = other RNA
tgtcttctctcctcccaaacaggattcaagtttccaaaaatggtcttggtacgcttcttagttttgctgacttgcacagtcacgtaagggtcactggatcctgttttgtccttggcttgtaggccctgggcacacaccacagtaatggtgatcttggctgaccatttggaggtgccatccagtacactctgcttcactgttttcatctgctgcacatgggcagctttgttcactgtgaagacgtcccggataacttcaaagatctctggcttatttcgctctcggatcttcatgcggtccttcatggccatgataatgttctgggtccggtcctcagctccatgtttacagctcttttctgcagcccgctgcaggcagtcagcattgagcagatcctggcacttctcatggcacttgactccacattcgctgcagcgcatgccctgccgggcaatgccccagagcaggccttcacactcatagcagtaggttggggtagtggccgtccagacctcaaagttatgaggagtggtgcacgaaatggggtagattaaggcctgcagggttttcttatacacgtgggatttcagctcttcgtccttaagagaagtgcgtgtagccattgcagaagtgattcctgccttccgagactggaccagtgacagatcactgacaagtggcagtggcttctttctgcgtaaatctggcatgctgtcaatgccatagagccctccggctggcccttccgggagccactgaggcagagaggggtcaccatcatctggaatctcctgcagctggagtcgaaccttggtaactgctcggatccaatgtgctctggcttgggtaaatggtgaagatgcattctcctcaggaaaactctcctggggacctaggaagtggtctttttgcagcaccagatctgggggagggtgggttgtggcatcttctttcatctccttgggttcacatgctgcctccttctctgcttgacctgtcacctccaagggtttctcttgttctccaaaacctgcttggccatctctggacaggctgtgagagctgtggcaagaatgaatcgagtccgtctcccgatggtcgtcatcttgttcgtgatactggtctagttcacttagctgagagcttccttgactcacattacaggaggagccatacctactgctgctggtggggctgatagcccgccgctctggataatcaaggtcataactttgcatagagtcattacaagagtcccgggaactgccttgaagtagcagctgctgtggcgatcgcaccggcacagggaactggtgcacagaagcgttgggctgggaagctgtatggtaaggaggtgggaagctgttgctggtctcactgcgatagtcactatctcggtcatcgacggcactatcagggtcttcaaaagtctgttgttctccccagcccaaataggtccagtgacaacactgggcggcagcagtgggcaatggcttcctctggctttcttcttgactagaatactcattgtcagctcccaaggcattgatttgctcccatttgtaggtccaatatctggcttcctcctctgggatatcaaaaggcaactcaaatcttgtatcaagcaaaattttatgaggagttgggtttctagttccacagatctcatcgtctttcattaacgtctctgcctctaatgtggaccattccccaggcccttcctcatccgactgacgaatagtcttcagcgcaatccacacagtccccaccatggtgtcccagatcagtcctttgttccatacctccacacttagacccaggtccaggcgactaatctcaaacatgaaatcctgttcccaggaaggctgatcaccacgaactgctacagttgtgctcttcacattctgtactttcagggtcacatatgtgttaaatttatctggtgaaccctggaatttggcccttttaacgcgcacgcagagcagtgacatggccgaggatcgggcaagcctctgccgcgccccagccgcgccggaccgctccctctttcctctcagcaggtgccgcgactgctctcgttaccggccccacgggtctggcagctcctcatggtcccggtcgcaggtagcgtcccgccgctgcctcggacccgccccaaatctcaccgtctgagcgaactccgggtagcggtgagtaccggccggcaggctggggactgggcgcggcacagcgacgccatcgctgggaggtaggagctgccgggact

SEQ ID NO: 19179 - RNA, 10477 nt, Homo sapiens
  source 1..10477: mol_type = other RNA
tgtcttctctcctcccaaacaggattcaagtttccaaaaatggtcttggtacgcttcttagttttgctgacttgcacagtcacgtaagggtcactggatcctgttttgtccttggcttgtaggccctgggcacacaccacagtaatggtgatcttggctgaccatttggaggtgccatccagtacactctgcttcactgttttcatctgctgcacatgggcagctttgttcactgtgaagacgtcccggataacttcaaagatctctggcttatttcgctctcggatcttcatgcggtccttcatggccatgataatgttctgggtccggtcctcagctccatgtttacagctcttttctgcagcccgctgcaggcagtcagcattgagcagatcctggcacttctcatggcacttgactccacattcgctgcagcgcatgccctgccgggcaatgccccagagcaggccttcacactcatagcagtaggttggggtagtggccgtccagacctcaaagttatgaggagtggtgcacgaaatggggtagattaaggcctgcagggttttcttatacacgtgggatttcagctcttcgtccttaagagaagtgcgtgtagccattgcagaagtgattcctgccttccgagactggaccagtgacagatcactgacaagtggcagtggcttctttctgcgtaaatctggcatgctgtcaatgccatagagccctccggctggcccttccgggagccactgaggcagagaggggtcaccatcatctggaatctcctgcagctggagtcgaaccttggtaactgctcggatccaatgtgctctggcttgggtaaatggtgaagatgcattctcctcaggaaaactctcctggggacctaggaagtggtctttttgcagcaccagatctgggggagggtgggttgtggcatcttctttcatctccttgggttcacatgctgcctccttctctgcttgacctgtcacctccaagggtttctcttgttctccaaaacctgcttggccatctctggacaggctgtgagagctgtggcaagaatgaatcgagtccgtctcccgatggtcgtcatcttgttcgtgatactggtctagttcacttagctgagagcttccttgactcacattacaggaggagccatacctactgctgctggtggggcttttgttggtcatgggctccttgatgtcattcagagtgactggctgctgtacattcaaatcagagtcagtactggcaggtactgcctcctcttcttgtttttctagctggtgaaatatctcagagacagtggagggttcttcctcatgtttccctgaaggacaggcggggctagacaggttggctttggtatcccagtgttctccagatgctgagatttcctgctggtttcccccttctccagaccctgaaagcccctgagcacagacctctggactggccaccagctgctcagaggtcccagagggctgagtgtagactttacctggctgagcactggccccagatatttgagaagacttcaaagctttgttagcctcactggagttaaggtcctgatcactgctagtaactaaaactggaggggaggattctgtaggcatttgttcagggacccctttgttctcttttggccatggaaatgaaagatctacctttccaaatcctagttttgaatcacttgctaatacactccctttcccctcactacttccctcaaatagagttgacaacttcttaaaactggacattaaaccagtctctgctgctctattgccagaggggagaggtgaggaaaagaaagagctcagtggtttcccatggttagtagcagaggatggcaaacgaagctttggccaagtggtcacatttgggatctcaaaacgtggtcttgactgctctgtttcctggggtactacaggtggatctttctgggcatgaattatctcacaactttctctggcagcaagcacagggtcctccagcagaggatgagaaaagtgcccttcggtttccagagtggtgctctggctcacacttgcatcattgaacagcatagtatcagtttctagtgaactggctggatgcagctccagtaagtcttggtttgtggaggcagtttgaatagctggctctggctcaagaggaagaggtggctgaatgggaggaggaagctcttcggcaatgcaggtaggatctggatgcaactgtgctggcagcgcaaagttctctgcttctaacgatgcctccgtgtctgtagcttgcaatatccccatgtctccttcatcactcagagacaatactccttgcccagtatcatcacccgagaaagaagatgtattaattgtttcagaacgttgaggttccagaatattttcaggagtattattgtcttccattttggttgttagtttaggatcatctgtcaagatatctgattctggctttgcactaaccacagtcattctacagtcactgagagtagattctgaacttagtgctgtaaaggcagcttctctcctttctggaggtactgatcctacagcatctctggaacaaccattttgaagccatgaagtagctgggagagatgattcttgtttgtatggctctggcttgggacttttgaaaattccaaataattcacctttgaggggctgagatgatacatcagaagcaagagagaaaaaggagtttttctttggagatttaggagaggagaaaagtccagagagtgttttgggaggttcaattaagctcccagagaaagatttcactttggtcacaaaccctgaaagcatgtctactgaagagcctaatgcaaatttgtcttcctctttatctgcatcttggttctgaaggttccctgcacaccctggctctggagaggaagaggctggctctaggatctgtggtaagacctcatcgggggccttttctaatggcaagttcactgggtcagtagtaaatttctcattttggtggcagttagtacaagtgtctaaatcattgaatttttcaattaactgtttagcatgtgaaaaagagttggacagtgagtcactggggaaggctttgtggttgaaagcctcttcttcatggggagctatcccaaggttctctgggccagtgaggaatgtttcagcctgtgcctgaaattctggtgaaggaggaataatgtctttttgcaattcattcatctggaaatccactgatgtccctggtacaatattggaactcagtttttcctgacagtccttgtctacactgagctcatctgcaagggaggtaacctcaatggtgttgttaatggaaatacaaggtgccatttgctgttcatgaactacttcttgggctatgctatctctatgaccactggaactttctctggtcattgtgctaccactctctacaaaaacatttgtcttcttacagggctgggaggtcactggaacaacagttgaaatgctttgtttttccccagaggtctcctttttttgatccaaaaaggacaagctgaagaaactaaaagtagaactactatgagaggcatccttcttaatgcttgagctagcagtggaaaaaaatgaaggaagtgtgaatagcccttctgcctgagatttggctcttggtagagtagcagaggctctgttctcagatttttcagatccagtgagaaaagaaaatatactctttttggttgataactctggttgagatgaagatgttgcagccatagagaaactccagtctttgtcagaaaaatgatcttgttcatttgaatttctcttgctcagggtatcaaaggatatttcattactttttgaaacttctgtcactgtagtcacaccactagtttctactgaagactccctggaagactctttgagactacttgttgaaaaagatgaattaggtgactgctggattagatggtctctgaatggtacctctttttcagtcaaatcattaccctggatccctctagttgattcctctaacctactgtcatcgatagtagtctgtttgttcagtcttctaactctagccttccctttagaggaaattggtgcagcaggaaagttcccagcaccctggctagctagctccataggagtaggacttgacctgacctcatccttaatagtcattgaagaaacagacgtattttcagttgtctgtataggagatacattggctttaaagaaatccccaagggtaccccaaaaatttgaaacaccagaagattctttcttttcttgaggtggtatcttgacatttgtatcaccaatcttttctaagtttggtgatccttctttattcacctgagtcttaaaaagattcaaaaatccagatgactgtttttcatttgctgtcatactaactgacgattcttcttgactgaagagtttcaatgaacttttaaataatgttttatcagactctttggatgactggccctggggaagctcataattctcacgctcatccccactatgctgaggtgcaggagaaactgaaatagagtctgttgtaatgatttcatcatcttttacacctgatttagcctgaggagttgtttggcttacctggaaaccagattttaacaaactttgctttttcacatggttgtttttatttaaagagaattcttgccttatatttttgatcaattctggatgctgaacattggatactatctgtctttctgaatccttaagaagacttttttccacatttggggagttaccctctaattgcttactcatgattaatgactgaaagccatcatttgtgagctctgctaaatctgactgctgattcactttctgcatggccaaagcctctaaggattcactcttatcaaacttcaaagtactaccaactgaggcacccaaaacagaaaatactgaagccactttgttcactaatgatgtctcttctgcttgttgtgagcctttagtcatattttcaggatgaaccaaagtggtaacttcttcaacagaagactgaagccaatggaaactggaaaggtgaactgatgaatcttcagctagaggctggtttttatctctctctataatttgatctctgcttgagacatgattactaatagtttggggctgatttctgagatctaatgtacattcagcgtcttcagaaccacacggcctttctttgaaagatctaaagtctcctttaaacttttgacgattatagcctgaaaaatctagtggctgatcgctttggtcacaacttgactctttaagtacttgtgaaaaggtttctaaatttagatacaatggttcctcacttcttggcaaagctaaagataaatcaagagggtcatcaattggttcctcttcaacataccaaaatatttcatcttccttatcaagtactttaaaactacaggcagaaataatgctgtcatccaacgtaatacttgatagaccatttgtctgtaaatcacaatccaaatactcttgataagaatcaggtataaataaatatgcatactgcccagtagaatcagtgagaagagaatagatatattgaccatcatgaaacatataatatccataatccccatcctctgatggccaccacactccatgttcaagacatgacaaccattcctggtactcataaccaaaacttgaaaaaacaaagttttcatccattcttaatgattcttgatcaactacggggcatgtagtcttttcatgatctgatgaagaacttaagtcaatgggtaattcttctagtgaattattagcctcattaattggaagaggaccagagtttccatataatgagttagctgcccacacatcacctcttaataagtaatcttcattaaatgctaactgattgaatgattcatatggtaagtcacaccaaatgacactgtttggatttgttctccactccaagatgtttgcattttgatctttttggcaaaaatttatcactgagttttctgagtcaagccacaagcaagcatcggctgatagaaatctattttgatttaacatataataaactggctgaagttttctggaatttttagacaaatcttttatgtcagagtcccattcaaaacagaaaggactgttcatctcttcaaaagcctgatagttgtttgatttattgagaatgttggtatttagtacaggtgaatttaacttgtttgaattttcatgtagttttgcctcaagaacatggtttggcatttgcctcttagccatagatttctccaaaaaacctagctgagcacttggagcacagtgaagtacaatgttctcagaggaggggtgatgcttttcactttgctggtttttctctgtaggggaacaataatgattatcatccccagcatcagataatggtatgttttctttaggtaataaggaggcttctatgaagctagaagtttcatgtttttcaacatggttcttcgggttctcagaagtcacacatgaagtagcagggacctcatccaaggataaatggttatctccattcaaactcttcatgttgcctaaagacatgaactttgcttcctctggtttatgatcaatcataccgctatttgatagcaggttaaatattccagagattaaacctggggtattattcttgtgatgggagtcatcatttttcaaatttaattcttgactagacaaattttcagcagaagaaaacctattaaacaggccagaaaggaagcttccttgggtatttttcttggaagtcttatctataacctcatcttcattaatttcattaaccaaagtggatttggaagtggtagaaatacactctaatgaagagtctgatgctactgaagatgctgcttgtataagattcttatcttctcctaaaggatctgaagttatatgttctttgggcacaactccagggatggctaagccatccctttcaaaattctgtcctgctgtgtggtcacttggatttaattcctctatattcccaaatttccccagatcattattaatatttgtaactgaatcagactttattatattaaatttggcatcttcaggactatttatttggtcattctgattaaattcctctgtactgtcaaatttccctagattatcctgagtatttggagctgaaccagattttattgaactaagtttggcatcttcaggacaatttacttggtcattcttattaaattcctttatactgtcaaacttctctagatcatcatgaatatttggaactgaactagattttattgaattaagtttggcatcttcaggacaatttatctggtcattctttttaaattcctctgtactgtcaaattttcctagatcactatgaatatttggaacagaactagattttattgaactatgtttggtatcttcatggcaattttttttgctctcctcatcagtggttactgctgagccacgtaaactctggtcattaacagtaaccttgctgtcagtgaaagaaaatttaaacaaaggaaaaatgcttcctttctcttttaactcctgttgcttttcagaatgaccaagacttctaaaaaatggaagatttagttttccactaaaggaaaaggaatgaccatctttcttagagcccctttctaaaccatcttcctccacctggcgaattttcacaggttctgacaaactttcctttgaacaagtctcaggggaagtgagcaaaaactggctaaatgattttctgagtggctcaaggaaatcatcattacctgtaactttgtcctcctctaatggctttgaaaatacctctttatttgcagttctactgccagctatacaaggatgtcctggagtatctttggcacatattttttgttgatctggtaaaagagacagatctatacagagtttttcttccaatagactctcatcatttttacttgcagaactaactaagtttgaaggttcactggttacttgggaggacaacaaattctcacttgtgggcatctggaaccagcccgtagtttcttcatcactcccatttaaagcaatgatgctactactgtaattgtcaagagtgccttcccttttatttaactccaaaccacactcaacaaagctttcttttcttggtggcttactctggtcatcatctttttttgtttcctccttttctgaaaagatcttcaatggatttaacctgctgaaaaccgactttataactgaactctgactctgtggagccaagtcctttgcaatactttctgttgtattctgaaagtataaactcccagttttattacccatgtgctcattttcagaggtttttctatgtctgtctatattcacattatcatctttttgagaggataatggagattgcatggaaagatccttccccaatactgccatggctctgggtttagatcccaaattaattgcctctatttgattaagagtttctgttttttctggaactaaggaaaccaacttttccacagagtttgttagatgctttgtgcctgaacccactttttctgtgagtgaactaaacaaagaaccaacagcacattgtactccagtcaactcagggaaagagatggccgtgtccttgtcattcttgacaatagttaaaggtggtatttgatccccaggcgttctctgttctgcatcaagagtactattttgtttatgtgattttttagtttttgaaagtgaaccaaatctattaatctcctcttccttctctgctaaatattctgacaccgtttctaccaaacactgaagctcatccattgtatcaatacggtcctccttgggctcctcaatagaggaaggggttatctcttctatagagcactcagacagatctccaagtgtttttgcatcacaattcatcctttgtaatggcaatgctgaatttgctacataatattcctcaggaaaatctccaatatggtggacattggatgaatgccatgttggtgactgtaaattttcctgcttatcagaaatgggggaacccagaagttcatcagaagtactactagtagaatcttcaagaatatctaatgaggtaaaattagtgacatgctggtttgagccagatgacttttcacagtgccttaaacaactggacagatcataatcatgactttccaacttaatgcgctgcatgccactcttaaccacaaatccatttttgtaggggtacaaaactgggtaccccatattttgtttcttttcagtatggcaaagggtacaattttcagtattagaatatgtacttttgtagttagtcttagtttcagatctctcaccatattgccttctttcactgtcttcaaaatgattgtataaggatttcttttttcttcttctatctagtgtatcatatttctgagcatacctgatagcccgccgctctggataatcaaggtcataactttgcatagagtcattacaagagtcccgggaactgccttgaagtagcagctgctgtggcgatcgcaccggcacagggaactggtgcacagaagcgttgggctgggaagctgtatggtaaggaggtgggaagctgttgctggtctcactgcgatagtcactatctcggtcatcgacggcactatcagggtcttcaaaagaacactgggcggcagcagtgggcaatggcttcctctggctttcttcttgactagaatactcattgtcagctcccaaggcattgatttgctcccatttgtaggtccaatatctggcttcctcctctgggatatcaaaaggcaactcaaatcttgtatcaagcaaaattttatgaggagttgggtttctagttccacagatctcatcgtctttcattaacgtctctgcctctaatgtggaccattccccaggcccttcctcatccgactgacgaatagtcttcagcgcaatccacacagtccccaccatggtgtcccagatcagtcctttgttccatacctccacacttagacccaggtccaggcgactaatctcaaacatgaaatcctgttcccaggaaggctgatcaccacgaactgctacagttgtgctcttcacattctgtactttcagggtcacatatgtgttaaatttatctggtgaaccctggaatttggcccttttaacgcgcacgcagagcagtgacatggccgaggatcgggcaagcctctgccgcgccccagccgcgccggaccgctccctctttcctctcagcaggtgccgcgactgctctcgttaccggccccacgggtctggcagctcctcatggtcccggtcgcaggtagcgtcccgccgctgcctcggacccgccccaaatctcaccgtctgagcgaactccgggtagcggtgagtaccggccggcaggctggggactgggcgcggcacagcgacgccatcgctgggaggtaggagctgccgggact

SEQ ID NO: 19180 - RNA, 1217 nt, Homo sapiens
  source 1..1217: mol_type = other RNA
tgtcttctctcctcccaaacaggattcaagtttccaaaaatggtcttggtacgcttcttagttttgctgacttgcacagtcacgtaagggtcactggatcctgttttgtccttggcttgtaggccctgggcacacaccacagtaatggtgatcttggctgaccatttggaggtgccatccagtacactctgcttcactgttttcatctgctgcacatgggcagctttgttcactgtgaagacgtcccggataacttcaaagatctctggcttatttcgctctcggatcttcatgcggtccttcatggccatgataatgttctgggtccggtcctcagctccatgtttacagctcttttctgcagcccgctgcaggcagtcagcattgagcagatcctggcacttctcatggcacttgactccacattcgctgcagcgcatgccctgccgggcaatgccccagagcaggccttcacactcatagcagtaggttggggtagtggccgtccagacctcaaagttatgaggagtggtgcacgaaatggggtagattaaggcctgcagggttttcttatacacgtgggatttcagctcttcgtccttaagagaagtgcgtgtagccattgcagaagtgattcctgccttccgagactggaccagtgacagatcactgacaagtggcagtggcttctttctgcgtaaatctggcatgctgtcaatgccatagagccctccggctggcccttccgggagccactgaggcagagaggggtcaccatcatctggaatctgaagggctcctcgcttttcttctcctgcagctggagtcgaaccttggtaactgctcggatccaatgtgctctggcttgggtaaatggtgaagatgcattctcctcaggaaaactctcctggggacctaggaagtggtctttttgcagcaccagatctgggggagggtgggttgtggcatcttctttcatctccttgggttcacatgctgcctccttctctgcttgacctgtcacctccaagggtttctcttgttctccaaaacctgcttggccatctctggacaggctgtgagagctgtggcaagaatgaatcgagtccgtctcccgatggtcgtcatcttgttcgtgatactggtctagttcacttagctgagagcttccttgactcacattacaggaggagccatacctactgctgctggtgggg

SEQ ID NO: 19181 - RNA, 3777 nt, Homo sapiens
  source 1..3777: mol_type = other RNA
tgtcttctctcctcccaaacaggattcaagtttccaaaaatggtcttggtacgcttcttagttttgctgacttgcacagtcacgtaagggtcactggatcctgttttgtccttggcttgtaggccctgggcacacaccacagtaatggtgatcttggctgaccatttggaggtgccatccagtacactctgcttcactgttttcatctgctgcacatgggcagctttgttcactgtgaagacgtcccggataacttcaaagatctctggcttatttcgctctcggatcttcatgcggtccttcatggccatgataatgttctgggtccggtcctcagctccatgtttacagctcttttctgcagcccgctgcaggcagtcagcattgagcagatcctggcacttctcatggcacttgactccacattcgctgcagcgcatgccctgccgggcaatgccccagagcaggccttcacactcatagcagtaggttggggtagtggccgtccagacctcaaagttatgaggagtggtgcacgaaatggggtagattaaggcctgcagggttttcttatacacgtgggatttcagctcttcgtccttaagagaagtgcgtgtagccattgcagaagtgattcctgccttccgagactggaccagtgacagatcactgacaagtggcagtggcttctttctgcgtaaatctggcatgctgtcaatgccatagagccctccggctggcccttccgggagccactgaggcagagaggggtcaccatcatctggaatctgaagggctcctcgcttttcttctgagtgtatgtcttctactgagagacggtttgccttctgtactagctcatgcagaagttttttctgccttagtcttttctctcttagaacattcttaaaattgttgatgcacttgttgaggtaaacggtctctgtacacacttgctctaggctcagtctgccctgcttgggagatccaggcctggaacaagtctcacttcccagacatggagccagagcaacacttggcaaggagttattagaagcaagagagaaggtgcttggatcctgaggggtttgctctccctgtgtggagacgccaactccaccagagaccacactgagcaagctttcactcccctgactcccagggctctccagtgagcaatcctgggcaccccctgaactcactgtcccaagaagtcgatcactgttctctgactgggaaccactctcattgctttccaggtcctcaggactgatggacccactgttctccagcttctgaaacacaccctgcagagcagaacgaaagtggtgaattgctcggcccagtttacttgtataaaacttgatttccacatcctcatcctcctgagagccacccagaacacaagaggacttgtcaaagacatccttgaggacgtgagcagcacattcctcctcttcattcaggtcaatatgaaccatgtcactgaaagtctcaggccctatgataatttcctccatcatgctgtcacagctcagagctgcaagccttctggacttgtctgccaaaaggtcctctagttcctttgagctcagaatatcgagcccagcttcgcagcccaggagcttgtcctctgcgtttattctctctgtcttcagtaacccagacaatgacaggcagctgctggcctcacttttatcgtggcagtcattttctggttttcctactttacatgcttcatgtttttggctgtactgtttgaaaaactgggacttcccagaagcctcctcttttgagattaatactagggcaggttcctcaaactgatggggggtagacagagaagcctttttctctgacagttcatcacagctgccactgataacttgagatgttcttgatgctccttttatttcatcccctagcttgggcacatcactttcctttgataaattgttcttgagtagaaagcaagggccttgctgctcaggggcctggtgctctctctgttgatcctgagccttcatctgatatgttcctgttatgggtcccctgtcccctgtttccatctgaagaactggttcatcctggtttaaagaagtctgactataatcctgatgttgttgttgaaaaaatgatatagactccttctggggattcttattaccctgtgggcagcttggttcttctctggtggcaattcggactcccacattctgcaagaggatggatttctgcaagatgaagtctctatgctctagatgggcaagcttcacaacagtgggcctaggggaaggggatgtgcctgccctgtaagcctttttaatgtacctgttgcactgcatgccattaacacaaaggtgcttggctagaaagctttccaccagttccatagtattttctccatcttgttcaggaagtccgtacaaatacagaatggcttcctcactgggtctgtccacgtggggttcctgggccttttcaccctcacacaccttggccagggaacaggtgctcacctgtaagccttctatttcactcagtactgagtctacacagctagagacttcatccacggaaccctggacttggctcaagtgctgctgcagctcagcaatctcagtctgaagacggctgatgccttgcagctctctgatgatgtattctactacatcccccaaaggttcccgctgttcacggctacagccttggccatggcctctggacaaaagggtcttggtttggttcctctctgagggctcctgacagcttgtggtaatgctgacagatgagggatcctgagaaccagaccctgaaacataggcagtggagcccagaggaagctggctgttgttctgctgcccaaagctgcaaagctgggccaggtccccatctctatctccaccaatggctaaggctgctgacccacagcaagggggcagggagttgtcctctggtaaggatccagcagggccagaggatttgctcttggtgccacacatggtctctgccttagccttatctggggaaagcctggaggagggtcccaaggtaaccatgatttcttcctctgactcttgcaacaatcgcttcattttctccctcagggtttgaggggttctctgcttcttcctcttatttctggtcaggatgcttaatagagattaccttggaaggcaacagcctgtcctgctcttttcagtttgtttctagcaattattgctggctgatgctttgggcttagcccacagtgctgcctggaatggccccatgtgtggcctccaaacctcgcacatgcccctggatcctggcttgatttatcctgtagcttgctgctgcaaccaaaataagggttaaggaaattaaaaaaaaaaattaaaaccatgaattctcaagttttagaaggcaaatgctgtctttaagaggaaatccatccaggagcactccttggtttgacagagaagccacaggacgaactttctgagccaaagcaccactgcttgcccaaccgacaaacagacccaaggagctaatattctcagttgcacccagctggctggctccacggcacaaagttgatgacagaaacaatgccctgcaaaaaaacccctcagtgaagggcttggcaggagtctcactggctgcaaacgtagaaatctaacctggtccacacctctctggcaagggggattctgagatcagcctgctgaaggcaacagcagccaaacttcaactggatgtggaattctaactcaatcgattctgggctttgagact

SEQ ID NO: 19182 - RNA, 7407 nt, Homo sapiens
  source 1..7407: mol_type = other RNA
tgtcttctctcctcccaaacaggattcaagtttccaaaaatggtcttggtacgcttcttagttttgctgacttgcacagtcacgtaagggtcactggatcctgttttgtccttggcttgtaggccctgggcacacaccacagtaatggtgatcttggctgaccatttggaggtgccatccagtacactctgcttcactgttttcatctgctgcacatgggcagctttgttcactgtgaagacgtcccggataacttcaaagatctctggcttatttcgctctcggatcttcatgcggtccttcatggccatgataatgttctgggtccggtcctcagctccatgtttacagctcttttctgcagcccgctgcaggcagtcagcattgagcagatcctggcacttctcatggcacttgactccacattcgctgcagcgcatgccctgccgggcaatgccccagagcaggccttcacactcatagcagtaggttggggtagtggccgtccagacctcaaagttatgaggagtggtgcacgaaatggggtagattaaggcctgcagggttttcttatacacgtgggatttcagctcttcgtccttaagagaagtgcgtgtagccattgcagaagtgattcctgccttccgagactggaccagtgacagatcactgacaagtggcagtggcttctttctgcgtaaatctggcatgctgtcaatgccatagagccctccggctggcccttccgggagccactgaggcagagaggggtcaccatcatctggaatctgaagggctcctcgcttttcttctgagtgtatgtcttctactgagagacggtttgccttctgtactagctcatgcagaagttttttctgccttagtcttttctctcttagaacattcttaaaattgttgatgcacttgttgaggtaaacggtctctgtacacacttgctctaggctcagtctgccctgcttgggagatccaggcctggaacaagtctcacttcccagacatggagccagagcaacacttggcaaggagttattagaagcaagagagaaggtgcttggatcctgaggggtttgctctccctgtgtggagacgccaactccaccagagaccacactgagcaagctttcactcccctgactcccagggctctccagtgagcaatcctgggcaccccctgaactcactgtcccaagaagtcgatcactgttctctgactgggaaccactctcattgctttccaggtcctcaggactgatggacccactgttctccagcttctgaaacacaccctgcagagcagaacgaaagtggtgaattgctcggcccagtttacttgtataaaacttgatttccacatcctcatcctcctgagagccacccagaacacaagaggacttgtcaaagacatccttgaggacgtgagcagcacattcctcctcttcattcaggtcaatatgaaccatgtcactgaaagtctcaggccctatgataatttcctccatcatgctgtcacagctcagagctgcaagccttctggacttgtctgccaaaaggtcctctagttcctttgagctcagaatatcgagcccagcttcgcagcccaggagcttgtcctctgcgtttattctctctgtcttcagtaacccagacaatgacaggcagctgctggcctcacttttatcgtggcagtcattttctggttttcctactttacatgcttcatgtttttggctgtactgtttgaaaaactgggacttcccagaagcctcctcttttgagattaatactagggcaggttcctcaaactgatggggggtagacagagaagcctttttctctgacagttcatcacagctgccactgataacttgagatgttcttgatgctccttttatttcatcccctagcttgggcacatcactttcctttgataaattgttcttgagtagaaagcaagggccttgctgctcaggggcctggtgctctctctgttgatcctgagccttcatctgatatgttcctgttatgggtcccctgtcccctgtttccatctgaagaactggttcatcctggtttaaagaagtctgactataatcctgatgttgttgttgaaaaaatgatatagactccttctggggattcttattaccctgtgggcagcttggttcttctctggtggcaattcggactcccacattctgcaagaggatggatttctgcaagatgaagtctctatgctctagatgggcaagcttcacaacagtgggcctaggggaaggggatgtgcctgccctgtaagcctttttaatgtacctgttgcactgcatgccattaacacaaaggtgcttggctagaaagctttccaccagttccatagtattttctccatcttgttcaggaagtccgtacaaatacagaatggcttcctcactgggtctgtccacgtggggttcctgggccttttcaccctcacacaccttggccagggaacaggtgctcacctgtaagccttctatttcactcagtactgagtctacacagctagagacttcatccacggaaccctggacttggctcaagtgctgctgcagctcagcaatctcagtctgaagacggctgatgccttgcagctctctgatgatgtattctactacatcccccaaaggttcccgctgttcacggctacagccttggccatggcctctggacaaaagggtcttggtttggttcctctctgagggctcctgacagcttgtggtaatgctgacagatgagggatcctgagaaccagaccctgaaacataggcagtggagcccagaggaagctggctgttgttctgctgcccaaagctgcaaagctgggccaggtccccatctctatctccaccaatggctaaggctgctgacccacagcaagggggcagggagttgtcctctggtaaggatccagcagggccagaggatttgctcttggtgccacacatggtctctgccttagccttatctggggaaagcctggaggagggtcccaaggtaaccatgatttcttcctctgactcttgcaacaatcgcttcattttctccctcagggtttgaggggttctctgcttcttcctcttatttctggtcaggatgcttaatagagattaccttggaaggcaacagcctgtcctgctcttttcagtttgtttctagcaattattgctggctgatgctttgggcttagcccacagtgctgcctggaatggccccatgtgtggcctccaaacctcgcacatgcccctggatcctggcttgatttatcctgtagcttgctgctgcaaccaaaataagggttaaggaaattaaaaaaaaaaattaaaaccatgaattctcaagttttagaaggcaaatgctgtctttaagaggaaatccatccaggagcactccttggtttgacagagaagccacaggacgaactttctgagccaaagcaccactgcttgcccaaccgacaaacagacccaaggagctaatattctcagttgcacccagctggctggctccacggcacaaagttgatgacagaaacaatgccctgcaaaaaaacccctcagtgaagggcttggcaggagtctcactggctgcaaacgtagaaatctaacctggtccacacctctctggcaagggggattctgagatcagcctgctgaaggcaacagcagccaaacttcaactggatgtggaattctaactcaatcgattctgggctttgagactgaggcagaaagcagggcagctcctgctcctgctgctgctcctcctcctctccagctgcttcctgcctgcaacctcccatagggcaccagccctcctcacacgttcctggcgcacacacccccttcccagcacactcacgcacacacaacccttgccagcaagctcactcacacacccttggtaagtgtctctcccttttgctaaatatagatcttactctctcccctcctccatttccttccctcgttcttctcctccctgctttcttttcccctatccacctctctcacatctgggctataggatataaacagacacagatggagacctatactttcaggagctcctagtctcagagggaagccggaacacagcatgccagccgtggaactgctggagcacaatacaaagggagtcttcccttctactgagacaagctctaagttggttggttggttggtttcgtgtatatataatctgttgtcagcatttggcaaagctgaaggataggtacagtgatcaagtgcagttaaaatcaaacagtgccatgttcttggagtagacatctattccagttcttactgaacaaccaccacaagagaatcaactggaaaataagagctccctcaggctatgccaaagcaacaacccgagagaaggaggggaagttaggtgagctgagatgaactctgtattgcagaagtctagaccaaagatggtttcagaatccagaattaggaacgaagtaacctaaagtgatatcaccatgaccaaaaagctgcctaaggttcagggccccttttatgaccccaaatttcataacccttctttgccaatggatgccctatctccctggagactcactagccaggtggctctcatgtgaccctaattcctaataattcaacaattctagttaggactcactgggaaattgaatgtccttatcttcaaagaacactcaagttgttcactgcaacataatgtccgagcacaagccaggaccccttgaagctctgtagcataaaatgccaaatacatgaaatgtgatatcccctttccactctgcaaccataggacatgaaaaacatcgcataatgaacctagataacctcagaatccttctcaatatagagctcgatcagccagtaacaatccagtgaagtcattcctcttctgactcccctgagcttgatcttaagagaaaaggccctcttcctccttaggccaacagtacgtgggcaagtttgatttacccagcatgcccaaaccaggctctcaaaccttgtgacttctgctgccctgcaacattcctcatggcaatccacaacagagtatggcctctttagcccacaaaccaggtagtcagtctatggggaccatcctaggatctgccattgcagaacaggcagccctttatggtagataaaacaagcatttaaattaagaatgatttgtttggcttatccaagatcctgagaagaaagggttgatttcagagccaacatgtgcctccctactgccttcttccaataacattgcttccccctcaaccaaggaagaaaatttagattccaagagatgctaaacaacccatttcttagccatccacctcattacacagccaacactaacagcagagcacatacctcctaacctagttgggagctggctagatgacagaagagataaggcctgacagcacaactataaccgcatctaaacacagaggaaaaaaataacttgaaaactgtcaagtttctgtggaagtcacagccaatttactgtggagtttcccatccttcagccaggagaaggaggtaaaaggtttaaaacaagaaatatagggaagattgattaaattagaattccctcccccaaatctgcagccactcataaagagcccagaacagtggctgtcactatcaggtttggtcaggcttcctaggctaaggagaagctcaaactttcaagagtgggaaagattccccagaggtaggaccctgctaaaagaacctacttcttcctgcctaattgacaaagtggccctaaggcctggctaaggcctccagatggcatttctgaggctaatggaacccaccctgtcttgtcacccaaacacatccagcccatttttctaagcagcttgggctttccagaaaaacaaaggctcaggcagtagaagacgtggttagcacatgaggcacaacaaatctgccatctccagttacaatcttcaaacttcacaggagagctcatgcagctttgaccacaaattacctttgtatctatccaccttcccatgttccagcaaaagcaagaaacagagtaagtggggaagtggcaaacagtcagtggaagctcttgtaaaagagcatggccccttctgccactgttctacagggcccacagagtgccagacaccacatggccaaaggacatcaggactcctcagtggactagctctttgggacaagcaggcaatttgttttgtgagccacatgggcaacaatgcagccccctcatcacagtggatctggccctggggaagcctgagtaggccgaaaggatggggtgctttttagaggtaagaaatagcacagcacccacctcagttgggaagcttcctcaaagtaggctgctcaggagctagctgggcagaactggaaaaacagattgggttaagaaggaaaaggcatttatccagaagctgtgaaatgctctgaacagacattctcaaggtctggttcccaatttaaatccttgcagggatcttcgcctagagacagatgagtcaagatggaaactcaacatgatacactgacactcacgcagagttgtgggaaggttcagacctgcaggagttctaaaggggagccgaatgggtgggttagtcagaaaaccacctggcatacaaaattcatcttcagctaaagcaactgagtggtgtcacagaaatactggaggagggcctcaccaatcacaattctccctactcatacaaaccagtctaagtctccctgacgtcagatacaactggtctagaagcaaagaatatgcctgctccaaacctggcctgccttttcaggtgtcaatgccagagacaggctgggtcaggaccagcaggtgcttaccttattgtccaatatcaacacagacgcagagtacaaaggatgggtgcggccaatatctatatcatgcaagagtcagcttgtgactgttttccttctctactgctgaggaaagccagaagcaacatgaaaaagctgacatatagtcacacagctgggatttatttcatgaggaagatgatttttctggtggctaagaaaagtcatttttcccgctgtagaatgatgccctccctacaccatggagaaagcatatgcagcagagaatgacgggcagcaggaggtaatcctgctccttccctgaggagcatgccatcctaggggagtgacaagcctggcagagatgtgctgactttactgatgcactaagacatagctgctttgttacctaaacagacccgacaagctgcaaggcaggccctaagagtcataaattgctgacaagtcttagtcctacaatcaggtcaaggaccatccctgattagcagaaacttgaaca

SEQ ID NO: 19183 - RNA, 1237 nt, Homo sapiens
  source 1..1237: mol_type = other RNA
tgtcttctctcctcccaaacaggattcaagtttccaaaaatggtcttggtacgcttcttagttttgctgacttgcacagtcacgtaagggtcactggatcctgttttgtccttggcttgtaggccctgggcacacaccacagtaatggtgatcttggctgaccatttggaggtgccatccagtacactctgcttcactgttttcatctgctgcacatgggcagctttgttcactgtgaagacgtcccggataacttcaaagatctctggcttatttcgctctcggatcttcatgcggtccttcatggccatgataatgttctgggtccggtcctcagctccatgtttacagctcttttctgcagcccgctgcaggcagtcagcattgagcagatcctggcacttctcatggcacttgactccacattcgctgcagcgcatgccctgccgggcaatgccccagagcaggccttcacactcatagcagtaggttggggtagtggccgtccagacctcaaagttatgaggagtggtgcacgaaatggggtagattaaggcctgcagggttttcttatacacgtgggatttcagctcttcgtccttaagagaagtgcgtgtagccattgcagaagtgattcctgccttccgagactggaccagtgacagatcactgacaagtggcagtggcttctttctgcgtaaatctggcatgctgtcaatgccatagagccctccggctggcccttccgggagccactgaggcagagaggggtcaccatcatctggaatcttgctgctgcaaccaaaataagggttaaggaaattaaaaaaaaaaattaaaaccatgaattctcaagttttagaaggcaaatgctgtctttaagaggaaatccatccaggagcactccttggtttgacagagaagccacaggacgaactttctgagccaaagcaccactgcttgcccaaccgacaaacagacccaaggagctaatattctcagttgcacccagctggctggctccacggcacaaagttgatgacagaaacaatgccctgcaaaaaaacccctcagtgaagggcttggcaggagtctcactggctgcaaacgtagaaatctaacctggtccacacctctctggcaagggggattctgagatcagcctgctgaaggcaacagcagccaaacttcaactggatgtggaattctaactcaatcgattctgggctttgagact

SEQ ID NO: 19184 - RNA, 1439 nt, Homo sapiens
  source 1..1439: mol_type = other RNA
tgtcttctctcctcccaaacaggattcaagtttccaaaaatggtcttggtacgcttcttagttttgctgacttgcacagtcacgtaagggtcactggatcctgttttgtccttggcttgtaggccctgggcacacaccacagtaatggtgatcttggctgaccatttggaggtgccatccagtacactctgcttcactgttttcatctgctgcacatgggcagctttgttcactgtgaagacgtcccggataacttcaaagatctctggcttatttcgctctcggatcttcatgcggtccttcatggccatgataatgttctgggtccggtcctcagctccatgtttacagctcttttctgcagcccgctgcaggcagtcagcattgagcagatcctggcacttctcatggcacttgactccacattcgctgcagcgcatgccctgccgggcaatgccccagagcaggccttcacactcatagcagtaggttggggtagtggccgtccagacctcaaagttatgaggagtggtgcacgaaatggggtagattaaggcctgcagggttttcttatacacgtgggatttcagctcttcgtccttaagagaagtgcgtgtagccattgcagaagtgattcctgccttccgagactggaccagtgacagatcactgacaagtggcagtggcttctttctgcgtaaatctggcatgctgtcaatgccatagagccctccggctggcccttccgggagccactgaggcagagaggggtcaccatcatctggaatcttgctgctgcaaccaaaataagggttaaggaaattaaaaaaaaaaattaaaaccatgaattctcaagttttagaaggcaaatgctgtctttaagaggaaatccatccaggagcactccttggtttgacagagaagccacaggacgaactttctgagccaaagcaccactgcttgcccaaccgacaaacagacccaaggagctaatattctcagttgcacccagctggctggctccacggcacaaagttgatgacagaaacaatgccctgcaaaaaaacccctcagtgaagggcttggcaggagtctcactggctgcaaacgtagaaatctaacctggtccacacctctctggcaagggggattctgagatcagcctgctgaaggcaacagcagccaaacttcaactggatgtggaattctaactcaatcgattctgggctttgagactgaggcagaaagcagggcagctcctgctcctgctgctgctcctcctcctctccagctgcttcctgcctgcaacctcccatagggcaccagccctcctcacacgttcctggcgcacacacccccttcccagcacactcacgcacacacaacccttgccagcaagctcactcacacacccttggtaagtgtctctcccttttgct

SEQ ID NO: 19185 - RNA, 2259 nt, Homo sapiens
  source 1..2259: mol_type = other RNA
tgtcttctctcctcccaaacaggattcaagtttccaaaaatggtcttggtacgcttcttagttttgctgacttgcacagtcacgtaagggtcactggatcctgttttgtccttggcttgtaggccctgggcacacaccacagtaatggtgatcttggctgaccatttggaggtgccatccagtacactctgcttcactgttttcatctgctgcacatgggcagctttgttcactgtgaagacgtcccggataacttcaaagatctctggcttatttcgctctcggatcttcatgcggtccttcatggccatgataatgttctgggtccggtcctcagctccatgtttacagctcttttctgcagcccgctgcaggcagtcagcattgagcagatcctggcacttctcatggcacttgactccacattcgctgcagcgcatgccctgccgggcaatgccccagagcaggccttcacactcatagcagtaggttggggtagtggccgtccagacctcaaagttatgaggagtggtgcacgaaatggggtagattaaggcctgcagggttttcttatacacgtgggatttcagctcttcgtccttaagagaagtgcgtgtagccattgcagaagtgattcctgccttccgagactggaccagtgacatagccagatcactgacaagtggcagtggcttctttctgcgtaaatctggcatgctgtcaatgccatagagccctccggctggcccttccgggagccactgaggcagagaggggtcaccatcatctggaatctgaagggctcctcgcttttcttctcctgcagctggagtcgaaccttggtaactgctcggatccaatgtgctctggcttgggtaaatggtgaagatgcattctcctcaggaaaactctcctggggacctaggaagtggtctttttgcagcaccagatctgggggagggtgggttgtggcatcttctttcatctccttgggttcacatgctgcctccttctctgcttgacctgtcacctccaagggtttctcttgttctccaaaacctgcttggccatctctggacaggctgtgagagctgtggcaagaatgaatcgagtccgtctcccgatggtcgtcatcttgttcgtgatactggtctagttcacttagctgagagcttccttgactcacattacaggaggagccatacctactgctgctggtggggctgatagcccgccgctctggataatcaaggtcataactttgcatagagtcattacaagagtcccgggaactgccttgaagtagcagctgctgtggcgatcgcaccggcacagggaactggtgcacagaagcgttgggctgggaagctgtatggtaaggaggtgggaagctgttgctggtctcactgcgatagtcactatctcggtcatcgacggcactatcagggtcttcaaaagaacactgggcggcagcagtgggcaatggcttcctctggctttcttcttgactagaatactcattgtcagctcccaaggcattgatttgctcccatttgtaggtccaatatctggcttcctcctctgggatatcaaaaggcaactcaaatcttgtatcaagcaaaattttatgaggagttgggtttctagttccacagatctcatcgtctttcattaacgtctctgcctctaatgtggaccattccccaggcccttcctcatccgactgacgaatagtcttcagcgcaatccacacagtccccaccatggtgtcccagatcagtcctttgttccatacctccacacttagacccaggtccaggcgactaatctcaaacatgaaatcctgttcccaggaaggctgatcaccacgaactgctacagttgtgctcttcacattctgtactttcagggtcacatatgtgttaaatttatctggtgaaccctggaatttggcccttttaacgcgcacgcagagcagtgacatggccgaggatcgggcaagcctctgccgcgccccagccgcgccggaccgctccctctttcctctcagcaggtgccgcgactgctctcgttaccggccccacgggtctggcagctcctcatggtcccggtcgcaggtagcgtcccgccgctgcctcggacccgccccaaatctcaccgtctgagcgaactccgggtagcggtgagtaccggccggcaggctggggactgggcgcggcacagcgacgccatcgctgggaggtaggagctgccgggact
